European Patent Application EP 4 520 821 A1 - sequence listing, part 11

SEQ ID NO: 15908 - RNA, 4177 nt, Homo sapiens
  source 1..4177: mol_type = other RNA
gctgggattacaggcatgagccatcacgcccggccaaagttttagaatttaagttattccaaaaaaaattttttttttcaaaaatacagactgcatccaattaaattctatgttaactggtaatgactaggtctaaaatgttaggtatttaccaataaatgacataaaataactcaacaacaaagggatttttttttttaagagatagggtctcactttatcactcaggtttggctgagggcagtggtgtgatcacagctcactgaagcctccaactcctgggctcaagtgatcctcccgcctcagtctaccagagtatattcttgaaagtaaaattacaaatgaaattcagcagtgttaaaaataagcccacttgcagacaattatcatttttcttcctttctttcctcactatctgtacttggcatatttcctacagtggctgtcttaaagaaaaaaaggaatccttcacaaatagtgtagccaaaaaagttggactaatatacaatgctatcagtaaagtattatatataaaatttataagtgctaaagtgtaattttgaaagacacttaagatactccttttttttttgagacaaggtctcagccctgtcgcccaggctggagtgcactagcacaacatcagctcactgcaacctccgcctcccaggttcaagcgattctcctgcctcagcctcccaagtagctgagactacaggcgcacgccagcatgtccagataattttttgtatttttagtagagatggggtttcaccatgttggccaggatggtctcaaatctcttgacctcgtgatctgcccatgtcggcttcccaaagtgttaggataacaggcatgagctaccgtgcccagcctacttaaaatattcttgaaatagctctccccacctccttttttttttttttttgagaatgagtttcactcgacacccaggctggagtgcagtggtgcgatcttggctcactgcaacctctgcctcccaggttcaagcgattatcctgcctcagcctcctgagtagctgggattacaaatgtgcaccaccacatctggctaattttttttttttttttttgtatttttagtagagacggggtttcaccaagttggcctggctggtctcgaacacctgacctcaattgatccacctgcctcggcctcccaaagtattataggcatgagccaccgagcccggccttttttgttttttgtttttttaaaggcagggttttgctctgttgcccaggctggagtgcagtggtgtgatcacagatcactgcagccttgacctctcctggtctcaagtgatcctcccacctcagccttcagaacagctgggactacaggtgtgtgtcaccatgcccagtaatttttttgtatatttgtagaggcagggtctcccaatgttgcctgggctggtctcaaactcctgggctcaagcaatccaccagctttggccttccaaagttctaggattatacgcatgagccactgtgccctgccccaatattttgttacttactagtgagactaaacacttttctaaaagtttgttagccatactatcctataaaagctgtttgttcatgtcttttgtccatttatctttttttttgtttttcttgagacagagtcttgctctgtggcccaggctggagtgcaggggtgcaatctcggctcactgcaagctccgcctcccaggttcaaatgattctcctgcctcagcctcctgagtagctgggattacaggcatgtgccaccatgcccagctaatttttttgtgtgtgtttttcagtagagatggggtttcaccatgttggccaggctgatctcgaattcctgacctcaggtgctccacccgcctcagcctcccaaagtactgggattacaggggtgagccaccgcacccggccaattttctgtatttttaatagagacagggtttcatcctgttggccaggctggcctcgaacttcggacctcaggtgatccacccgcctcgacctcccaaagtgctgggattacaggtgtgggccaccacacccagccaatttttttgtatttttagtagagacagggtttcatcatgttggccaggctggtcgcaaactcctgacctcaggtgatccacccgcctcagcatcccaaagtgctgggattacaggcatgagccaccactcccggccaatgttttgtatttttagtagagatggggtttcatcatgttggccagactggtctcaaactctggacctcaggtgatccacctgcctcagcctcccaaagtgtagggattacaggtgtgagccaccgcgcccagcctatgtttctattttatacatattcaacaaacatgattccccaacttctgcaaaataatttctttttcaagaacattgattttagagctcacactaagaaaaagaatacaaaaataatggcatagaaagtgaaaaaacaaaaataaaaagtagaaagctaaagtttcccattaaaatgatcaatatactgtgcagtaagtcaaatgtgtacaatgaattaagaaaatatgatatataaaaatccaaatttacaaaattaagtacaaataggtgtttatattacaaagtgatactggtttataaaaggattcaacatagattttttttaaatggttgttttcctcaatcaatttaacaatgattttaaatgtataaaattttaatatctctttgagacagtgatccaagcttcttcccttgatgatgttaccagttcatactttgtttcaataacctgtccctccacagaaagtaggtgcagtctcttcaccaatacactaagaagtactgtggtcaccatatatgcaaacctcaactctggacactcctgtgtgcctgagaatccaagtgaggaaaaagttttcattactaattcatcatcaaaccgatctggatcaaacttgtgtggagatggccaagtattaggatcctgaagtaccacaccaagggcataaaggacgagggtctctctaggaataataaatcggtcaatttttccttcaatatcttgaagctgggcagaaactggagtcagtttggcagttcgaacagtttcacaaagcacatgctgacaatatctgagctgctcaattttctctggagtaacaggaccatttccaaaaacttggtttatctcttcatataattttttttgaacttcttcagaggtggttaaaaaacagattgcccaggtacacaattttgcagttattatgcaactggccagagaaaatatcatactgtcttctaggatctgttggtcattaaggttcccttgtactaaggagtcaatgaaaatatgttgactgaagttccttccttttcgttcttttatgatgttccttaaaacagactccagttgcatgagggcatcttcatattgttttttccgagtcatgtttttatcaagtgacccatctagaaagccttttccaatctcagaccaaacctgaaaataggtaaatatacataatgtgccatgattcttctggaagcgaatgacttcctgatcatcttcaaatgtactacccattaccatctgtgtaacagacttcatagcaaaaccaagcatatgctggctgaggggcacgtgctgggtctctgggtaggagagccatttatctaataattcttctgaaagctttaggaggagggcaaagttactcttcagagaatcagtcacaccattttcatacaattttttcctcatgtggttttcactcacactgccaccaccagattgataccttaataatgacttcagcatggtttcaaaagggtccgatgtcttattgggattgatatgctgcttcagtacatcaacagtgcccaaactaaccacgaggcgcctgccaaaccagaaggagaccacaggcccatatctctcatgcaaattaaccaggaactcatgcaaacttccactattcacaatatctggaagattaccatctttttcttcagttggagtaatccctggaattcctgcagcttgtctggaagccggatagaggtagagcacggctcccaccaacgccagcaagaaggtaacggcgaagatcgcgaagtccaacatggttctgccgcccagggagccacgtctcggatcggccgctccagc

SEQ ID NO: 15909 - RNA, 3880 nt, Homo sapiens
  source 1..3880: mol_type = other RNA
gctgggattacaggcatgagccatcacgcccggccaaagttttagaatttaagttattccaaaaaaaattttttttttcaaaaatacagactgcatccaattaaattctatgttaactggtaatgactaggtctaaaatgttaggtatttaccaataaatgacataaaataactcaacaacaaagggatttttttttttaagagatagggtctcactttatcactcaggtttggctgagggcagtggtgtgatcacagctcactgaagcctccaactcctgggctcaagtgatcctcccgcctcagtctaccagagtatattcttgaaagtaaaattacaaatgaaattcagcagtgttaaaaataagcccacttgcagacaattatcatttttcttcctttctttcctcactatctgtacttggcatatttcctacagtggctgtcttaaagaaaaaaaggaatccttcacaaatagtgtagccaaaaaagttggactaatatacaatgctatcagtaaagtattatatataaaatttataagtgctaaagtgtaattttgaaagacacttaagatactccttttttttttgagacaaggtctcagccctgtcgcccaggctggagtgcactagcacaacatcagctcactgcaacctccgcctcccaggttcaagcgattctcctgcctcagcctcccaagtagctgagactacaggcgcacgccagcatgtccagataattttttgtatttttagtagagatggggtttcaccatgttggccaggatggtctcaaatctcttgacctcgtgatctgcccatgtcggcttcccaaagtgttaggataacaggcatgagctaccgtgcccagcctacttaaaatattcttgaaatagctctccccacctccttttttttttttttttgagaatgagtttcactcgacacccaggctggagtgcagtggtgcgatcttggctcactgcaacctctgcctcccaggttcaagcgattatcctgcctcagcctcctgagtagctgggattacaaatgtgcaccaccacatctggctaattttttttttttttttttgtatttttagtagagacggggtttcaccaagttggcctggctggtctcgaacacctgacctcaattgatccacctgcctcggcctcccaaagtattataggcatgagccaccgagcccggccttttttgttttttgtttttttaaaggcagggttttgctctgttgcccaggctggagtgcagtggtgtgatcacagatcactgcagccttgacctctcctggtctcaagtgatcctcccacctcagccttcagaacagctgggactacaggtgtgtgtcaccatgcccagtaatttttttgtatatttgtagaggcagggtctcccaatgttgcctgggctggtctcaaactcctgggctcaagcaatccaccagctttggccttccaaagttctaggattatacgcatgagccactgtgccctgccccaatattttgttacttactagtgagactaaacacttttctaaaagtttgttagccatactatcctataaaagctgtttgttcatgtcttttgtccatttatctttttttttgtttttcttgagacagagtcttgctctgtggcccaggctggagtgcaggggtgcaatctcggctcactgcaagctccgcctcccaggttcaaatgattctcctgcctcagcctcctgagtagctgggattacaggcatgtgccaccatgcccagctaatttttttgtgtgtgtttttcagtagagatggggtttcaccatgttggccaggctgatctcgaattcctgacctcaggtgctccacccgcctcagcctcccaaagtactgggattacaggggtgagccaccgcacccggccaattttctgtatttttaatagagacagggtttcatcctgttggccaggctggcctcgaacttcggacctcaggtgatccacccgcctcgacctcccaaagtgctgggattacaggtgtgggccaccacacccagccaatttttttgtatttttagtagagacagggtttcatcatgttggccaggctggtcgcaaactcctgacctcaggtgatccacccgcctcagcatcccaaagtgctgggattacaggcatgagccaccactcccggccaatgttttgtatttttagtagagatggggtttcatcatgttggccagactggtctcaaactctggacctcaggtgatccacctgcctcagcctcccaaagtgtagggattacaggtgtgagccaccgcgcccagcctatgtttctattttatacatattcaacaaacatgattccccaacttctgcaaaataatttctttttcaagaacattgattttagagctcacactaagaaaaagaatacaaaaataatggcatagaaagtgaaaaaacaaaaataaaaagtagaaagctaaagtttcccattaaaatgatcaatatactgtgcagtaagtcaaatgtgtacaatgaattaagaaaatatgatatataaaaatccaaatttacaaaattaagtacaaataggtgtttatattacaaagtgatactggtttataaaaggattcaacatagattttttttaaatggttgttttcctcaatcaatttaacaatgattttaaatgtataaaattttaatatctctttgagacagtgatccaagcttcttcccttgatgatgttaccagttcatactttgtttcaataacctgtccctccacagaaagtaggtgcagtctcttcaccaatacactaagaagtactgtggtcaccatatatgcaaacctcaactctggacactcctgtgtgcctgagaatccaagtgaggaaaaagttttcattactaattcatcatcaaaccgatctggatcaaacttgtgtggagatggccaagtattaggatcctgaagtaccacaccaagggcataaaggacgagggtctctctaggaataataaatcggtcaatttttccttcaatatcttgaagctgggcagaaactggagtcagtttggcagttcgaacagtttcacaaagcacatgctgacaatatctgagctgctcaattttctctggagtaacaggaccatttccaaaaacttggtttatctcttcatataattttttttgaacttcttcagaggtggttaaaaaacagattgcccaggtacacaattttgcagttattatgcaactggccagagaaaatatcatactgtcttctaggatctgttggtcattaaggttcccttgtactaaggagtcaatgaaaatatgttgactgaagttccttccttttcgttcttttatgatgttccttaaaacagactccagttgcatgagggcatcttcatattgttttttccgagtcatgtttttatcaagtgacccatctagaaagccttttccaatctcagaccaaactgtgccatgattcttctggaagcgaatgacttcctgatcatcttcaaatgtactacccattaccatctgtgtaacagacttcatagcaaaaccaagcatatgctggctgaggggcacgtgctgggtctctgggtaggagagccatttatctaataattcttctgaaagcttaataatgacttcagcatggtttcaaaagggtccgttttcttcagttggagtaatccctggaattcctgcagcttgtctggaagccggatagaggtagagcacggctcccaccaacgccagcaagaaggtaacggcgaagatcgcgaagtccaacatggttctgccgcccagggagccacgtctcggatcggccgctccagc

SEQ ID NO: 15910 - RNA, 4153 nt, Homo sapiens
  source 1..4153: mol_type = other RNA
gctgggattacaggcatgagccatcacgcccggccaaagttttagaatttaagttattccaaaaaaaattttttttttcaaaaatacagactgcatccaattaaattctatgttaactggtaatgactaggtctaaaatgttaggtatttaccaataaatgacataaaataactcaacaacaaagggatttttttttttaagagatagggtctcactttatcactcaggtttggctgagggcagtggtgtgatcacagctcactgaagcctccaactcctgggctcaagtgatcctcccgcctcagtctaccagagtatattcttgaaagtaaaattacaaatgaaattcagcagtgttaaaaataagcccacttgcagacaattatcatttttcttcctttctttcctcactatctgtacttggcatatttcctacagtggctgtcttaaagaaaaaaaggaatccttcacaaatagtgtagccaaaaaagttggactaatatacaatgctatcagtaaagtattatatataaaatttataagtgctaaagtgtaattttgaaagacacttaagatactccttttttttttgagacaaggtctcagccctgtcgcccaggctggagtgcactagcacaacatcagctcactgcaacctccgcctcccaggttcaagcgattctcctgcctcagcctcccaagtagctgagactacaggcgcacgccagcatgtccagataattttttgtatttttagtagagatggggtttcaccatgttggccaggatggtctcaaatctcttgacctcgtgatctgcccatgtcggcttcccaaagtgttaggataacaggcatgagctaccgtgcccagcctacttaaaatattcttgaaatagctctccccacctccttttttttttttttttgagaatgagtttcactcgacacccaggctggagtgcagtggtgcgatcttggctcactgcaacctctgcctcccaggttcaagcgattatcctgcctcagcctcctgagtagctgggattacaaatgtgcaccaccacatctggctaattttttttttttttttttgtatttttagtagagacggggtttcaccaagttggcctggctggtctcgaacacctgacctcaattgatccacctgcctcggcctcccaaagtattataggcatgagccaccgagcccggccttttttgttttttgtttttttaaaggcagggttttgctctgttgcccaggctggagtgcagtggtgtgatcacagatcactgcagccttgacctctcctggtctcaagtgatcctcccacctcagccttcagaacagctgggactacaggtgtgtgtcaccatgcccagtaatttttttgtatatttgtagaggcagggtctcccaatgttgcctgggctggtctcaaactcctgggctcaagcaatccaccagctttggccttccaaagttctaggattatacgcatgagccactgtgccctgccccaatattttgttacttactagtgagactaaacacttttctaaaagtttgttagccatactatcctataaaagctgtttgttcatgtcttttgtccatttatctttttttttgtttttcttgagacagagtcttgctctgtggcccaggctggagtgcaggggtgcaatctcggctcactgcaagctccgcctcccaggttcaaatgattctcctgcctcagcctcctgagtagctgggattacaggcatgtgccaccatgcccagctaatttttttgtgtgtgtttttcagtagagatggggtttcaccatgttggccaggctgatctcgaattcctgacctcaggtgctccacccgcctcagcctcccaaagtactgggattacaggggtgagccaccgcacccggccaattttctgtatttttaatagagacagggtttcatcctgttggccaggctggcctcgaacttcggacctcaggtgatccacccgcctcgacctcccaaagtgctgggattacaggtgtgggccaccacacccagccaatttttttgtatttttagtagagacagggtttcatcatgttggccaggctggtcgcaaactcctgacctcaggtgatccacccgcctcagcatcccaaagtgctgggattacaggcatgagccaccactcccggccaatgttttgtatttttagtagagatggggtttcatcatgttggccagactggtctcaaactctggacctcaggtgatccacctgcctcagcctcccaaagtgtagggattacaggtgtgagccaccgcgcccagcctatgtttctattttatacatattcaacaaacatgattccccaacttctgcaaaataatttctttttcaagaacattgattttagagctcacactaagaaaaagaatacaaaaataatggcatagaaagtgaaaaaacaaaaataaaaagtagaaagctaaagtttcccattaaaatgatcaatatactgtgcagtaagtcaaatgtgtacaatgaattaagaaaatatgatatataaaaatccaaatttacaaaattaagtacaaataggtgtttatattacaaagtgatactggtttataaaaggattcaacatagattttttttaaatggttgttttcctcaatcaatttaacaatgattttaaatgtataaaattttaatatctctttgagacagtgatccaagcttcttcccttgatgatgttaccagttcatactttgtttcaataacctgtccctccacagaaagtaggtgcagtctcttcaccaatacactaagaagtactgtggtcaccatatatgcaaacctcaactctggacactcctgtgtgcctgagaatccaagtgaggaaaaagttttcattactaattcatcatcaaaccgatctggatcaaacttgtgtggagatggccaagtattaggatcctgaagtaccacaccaagggcataaaggacgagggtctctctaggaataataaatcggtcaatttttccttcaatatcttgaagctgggcagaaactggagtcagtttggcagttcgaacagtttcacaaagcacatgctgacaatatctgagctgctcaattttctctggagtaacaggaccatttccaaaaacttggtttatctcttcatataattttttttgaacttcttcagaggtggttaaaaaacagattgcccaggtacacaattttgcagttattatgcaactggccagagaaaatatcatactgtcttctaggatctgttggtcattaaggttcccttgtactaaggagtcaatgaaaatatgttgactgaagttccttccttttcgttcttttatgatgttccttaaaacagactccagttgcatgagggcatcttcatattgttttttccgagtcatgtttttatcaagtgacccatctagaaagccttttccaatctcagaccaaactgtgccatgattcttctggaagcgaatgacttcctgatcatcttcaaatgtactacccattaccatctgtgtaacagacttcatagcaaaaccaagcatatgctggctgaggggcacgtgctgggtctctgggtaggagagccatttatctaataattcttctgaaagctttaggaggagggcaaagttactcttcagagaatcagtcacaccattttcatacaattttttcctcatgtggttttcactcacactgccaccaccagattgataccttaataatgacttcagcatggtttcaaaagggtccgatgtcttattgggattgatatgctgcttcagtacatcaacagtgcccaaactaaccacgaggcgcctgccaaaccagaaggagaccacaggcccatatctctcatgcaaattaaccaggaactcatgcaaacttccactattcacaatatctggaagattaccatctttttcttcagttggagtaatccctggaattcctgcagcttgtctggaagccggatagaggtagagcacggctcccaccaacgccagcaagaaggtaacggcgaagatcgcgaagtccaacatggttctgccgcccagggagccacgtctcggatcggccgctccagc

SEQ ID NO: 15911 - RNA, 3936 nt, Homo sapiens
  source 1..3936: mol_type = other RNA
gctgggattacaggcatgagccatcacgcccggccaaagttttagaatttaagttattccaaaaaaaattttttttttcaaaaatacagactgcatccaattaaattctatgttaactggtaatgactaggtctaaaatgttaggtatttaccaataaatgacataaaataactcaacaacaaagggatttttttttttaagagatagggtctcactttatcactcaggtttggctgagggcagtggtgtgatcacagctcactgaagcctccaactcctgggctcaagtgatcctcccgcctcagtctaccagagtatattcttgaaagtaaaattacaaatgaaattcagcagtgttaaaaataagcccacttgcagacaattatcatttttcttcctttctttcctcactatctgtacttggcatatttcctacagtggctgtcttaaagaaaaaaaggaatccttcacaaatagtgtagccaaaaaagttggactaatatacaatgctatcagtaaagtattatatataaaatttataagtgctaaagtgtaattttgaaagacacttaagatactccttttttttttgagacaaggtctcagccctgtcgcccaggctggagtgcactagcacaacatcagctcactgcaacctccgcctcccaggttcaagcgattctcctgcctcagcctcccaagtagctgagactacaggcgcacgccagcatgtccagataattttttgtatttttagtagagatggggtttcaccatgttggccaggatggtctcaaatctcttgacctcgtgatctgcccatgtcggcttcccaaagtgttaggataacaggcatgagctaccgtgcccagcctacttaaaatattcttgaaatagctctccccacctccttttttttttttttttgagaatgagtttcactcgacacccaggctggagtgcagtggtgcgatcttggctcactgcaacctctgcctcccaggttcaagcgattatcctgcctcagcctcctgagtagctgggattacaaatgtgcaccaccacatctggctaattttttttttttttttttgtatttttagtagagacggggtttcaccaagttggcctggctggtctcgaacacctgacctcaattgatccacctgcctcggcctcccaaagtattataggcatgagccaccgagcccggccttttttgttttttgtttttttaaaggcagggttttgctctgttgcccaggctggagtgcagtggtgtgatcacagatcactgcagccttgacctctcctggtctcaagtgatcctcccacctcagccttcagaacagctgggactacaggtgtgtgtcaccatgcccagtaatttttttgtatatttgtagaggcagggtctcccaatgttgcctgggctggtctcaaactcctgggctcaagcaatccaccagctttggccttccaaagttctaggattatacgcatgagccactgtgccctgccccaatattttgttacttactagtgagactaaacacttttctaaaagtttgttagccatactatcctataaaagctgtttgttcatgtcttttgtccatttatctttttttttgtttttcttgagacagagtcttgctctgtggcccaggctggagtgcaggggtgcaatctcggctcactgcaagctccgcctcccaggttcaaatgattctcctgcctcagcctcctgagtagctgggattacaggcatgtgccaccatgcccagctaatttttttgtgtgtgtttttcagtagagatggggtttcaccatgttggccaggctgatctcgaattcctgacctcaggtgctccacccgcctcagcctcccaaagtactgggattacaggggtgagccaccgcacccggccaattttctgtatttttaatagagacagggtttcatcctgttggccaggctggcctcgaacttcggacctcaggtgatccacccgcctcgacctcccaaagtgctgggattacaggtgtgggccaccacacccagccaatttttttgtatttttagtagagacagggtttcatcatgttggccaggctggtcgcaaactcctgacctcaggtgatccacccgcctcagcatcccaaagtgctgggattacaggcatgagccaccactcccggccaatgttttgtatttttagtagagatggggtttcatcatgttggccagactggtctcaaactctggacctcaggtgatccacctgcctcagcctcccaaagtgtagggattacaggtgtgagccaccgcgcccagcctatgtttctattttatacatattcaacaaacatgattccccaacttctgcaaaataatttctttttcaagaacattgattttagagctcacactaagaaaaagaatacaaaaataatggcatagaaagtgaaaaaacaaaaataaaaagtagaaagctaaagtttcccattaaaatgatcaatatactgtgcagtaagtcaaatgtgtacaatgaattaagaaaatatgatatataaaaatccaaatttacaaaattaagtacaaataggtgtttatattacaaagtgatactggtttataaaaggattcaacatagattttttttaaatggttgttttcctcaatcaatttaacaatgattttaaatgtataaaattttaatatctctttgagacagtgatccaagcttcttcccttgatgatgttaccagttcatactttgtttcaataacctgtccctccacagaaagtaggtgcagtctcttcaccaatacactaagaagtactgtggtcaccatatatgcaaacctcaactctggacactcctgtgtgcctgagaatccaagtgaggaaaaagttttcattactaattcatcatcaaaccgatctggatcaaacttgtgtggagatggccaagtattaggatcctgaagtaccacaccaagggcataaaggacgagggtctctctaggaataataaatcggtcaatttttccttcaatatcttgaagctgggcagaaactggagtcagtttggcagttcgaacagtttcacaaagcacatgctgacaatatctgagctgctcaattttctctggagtaacaggaccatttccaaaaacttggtttatctcttcatataattttttttgaacttcttcagaggtggttaaaaaacagattgcccaggtacacaattttgcagttattatgcaactggccagagaaaatatcatactgtcttctaggatctgttggtcattaaggttcccttgtactaaggagtcaatgaaaatatgttgactgaagttccttccttttcgttcttttatgatgttccttaaaacagactccagttgcatgagggcatcttcatattgttttttccgagtcatgtttttatcaagtgacccatctagaaagccttttccaatctcagaccaaactgtgccatgattcttctggaagcgaatgacttcctgatcatcttcaaatgtactacccattaccatctgtgtaacagacttcatagcaaaaccaagcatatgctggctgaggggcacgtgctgggtctctgggtaggagagccatttatctaataattcttctgaaagctttaggaggagggcaaagttactcttcagagaatcagtcacaccattttcatacaattttttcctcatgtggttttcactcacactgccaccaccagattgataccttaataatgacttcagcatggtttcaaaagggtccgcggatagaggtagagcacggctcccaccaacgccagcaagaaggtaacggcgaagatcgcgaagtccaacatggttctgccgcccagggagccacgtctcggatcggccgctccagc

SEQ ID NO: 15912 - RNA, 4705 nt, Homo sapiens
  source 1..4705: mol_type = other RNA
gctgggattacaggcatgagccatcacgcccggccaaagttttagaatttaagttattccaaaaaaaattttttttttcaaaaatacagactgcatccaattaaattctatgttaactggtaatgactaggtctaaaatgttaggtatttaccaataaatgacataaaataactcaacaacaaagggatttttttttttaagagatagggtctcactttatcactcaggtttggctgagggcagtggtgtgatcacagctcactgaagcctccaactcctgggctcaagtgatcctcccgcctcagtctaccagagtatattcttgaaagtaaaattacaaatgaaattcagcagtgttaaaaataagcccacttgcagacaattatcatttttcttcctttctttcctcactatctgtacttggcatatttcctacagtggctgtcttaaagaaaaaaaggaatccttcacaaatagtgtagccaaaaaagttggactaatatacaatgctatcagtaaagtattatatataaaatttataagtgctaaagtgtaattttgaaagacacttaagatactccttttttttttgagacaaggtctcagccctgtcgcccaggctggagtgcactagcacaacatcagctcactgcaacctccgcctcccaggttcaagcgattctcctgcctcagcctcccaagtagctgagactacaggcgcacgccagcatgtccagataattttttgtatttttagtagagatggggtttcaccatgttggccaggatggtctcaaatctcttgacctcgtgatctgcccatgtcggcttcccaaagtgttaggataacaggcatgagctaccgtgcccagcctacttaaaatattcttgaaatagctctccccacctccttttttttttttttttgagaatgagtttcactcgacacccaggctggagtgcagtggtgcgatcttggctcactgcaacctctgcctcccaggttcaagcgattatcctgcctcagcctcctgagtagctgggattacaaatgtgcaccaccacatctggctaattttttttttttttttttgtatttttagtagagacggggtttcaccaagttggcctggctggtctcgaacacctgacctcaattgatccacctgcctcggcctcccaaagtattataggcatgagccaccgagcccggccttttttgttttttgtttttttaaaggcagggttttgctctgttgcccaggctggagtgcagtggtgtgatcacagatcactgcagccttgacctctcctggtctcaagtgatcctcccacctcagccttcagaacagctgggactacaggtgtgtgtcaccatgcccagtaatttttttgtatatttgtagaggcagggtctcccaatgttgcctgggctggtctcaaactcctgggctcaagcaatccaccagctttggccttccaaagttctaggattatacgcatgagccactgtgccctgccccaatattttgttacttactagtgagactaaacacttttctaaaagtttgttagccatactatcctataaaagctgtttgttcatgtcttttgtccatttatctttttttttgtttttcttgagacagagtcttgctctgtggcccaggctggagtgcaggggtgcaatctcggctcactgcaagctccgcctcccaggttcaaatgattctcctgcctcagcctcctgagtagctgggattacaggcatgtgccaccatgcccagctaatttttttgtgtgtgtttttcagtagagatggggtttcaccatgttggccaggctgatctcgaattcctgacctcaggtgctccacccgcctcagcctcccaaagtactgggattacaggggtgagccaccgcacccggccaattttctgtatttttaatagagacagggtttcatcctgttggccaggctggcctcgaacttcggacctcaggtgatccacccgcctcgacctcccaaagtgctgggattacaggtgtgggccaccacacccagccaatttttttgtatttttagtagagacagggtttcatcatgttggccaggctggtcgcaaactcctgacctcaggtgatccacccgcctcagcatcccaaagtgctgggattacaggcatgagccaccactcccggccaatgttttgtatttttagtagagatggggtttcatcatgttggccagactggtctcaaactctggacctcaggtgatccacctgcctcagcctcccaaagtgtagggattacaggtgtgagccaccgcgcccagcctatgtttctattttatacatattcaacaaacatgattccccaacttctgcaaaataatttctttttcaagaacattgattttagagctcacactaagaaaaagaatacaaaaataatggcatagaaagtgaaaaaacaaaaataaaaagtagaaagctaaagtttcccattaaaatgatcaatatactgtgcagtaagtcaaatgtgtacaatgaattaagaaaatatgatatataaaaatccaaatttacaaaattaagtacaaataggtgtttatattacaaagtgatactggtttataaaaggattcaacatagattttttttaaatggttgttttcctcaatcaatttaacaatgattttaaatgtataaaattttaatatctctttgagacagtgatccaagcttcttcccttgatgatgttaccagttcatactttgtttcaataacctgtccctccacagaaagtaggtgcagtctcttcaccaatacactaagaagtactgtggtcaccatatatgcaaacctcaactctggacactcctgtgtgcctgagaatccaagtgaggaaaaagttttcattactaattcatcatcaaaccgatctggatcaaacttgtgtggagatggccaagtattaggatcctgaagtaccacaccaagggcataaaggacgagggtctctctaggaataataaatcggtcaatttttccttcaatatcttgaagctgggcagaaactggagtcagtttggcagttcgaacagtttcacaaagcacatgctgacaatatctgagctgctcaattttctctggagtaacaggaccatttccaaaaacttggtttatctcttcatataattttttttgaacttcttcagaggtggttaaaaaacagattgcccaggtacacaattttgcagttattatgcaactggccagagaaaatatcatactgtcttctaggatctgttggtcattaaggttcccttgtactaaggagtcaatgaaaatatgttgactgaagttccttccttttcgttcttttatgatgttccttaaaacagactccagttgcatgagggcatcttcatattgttttttccgagtcatgtttttatcaagtgacccatctagaaagccttttccaatctcagaccaaactgtgccatgattcttctggaagcgaatgacttcctgatcatcttcaaatgtactacccattaccatctgtgtaacagacttcatagcaaaaccaagcatatgctggctgaggggcacgtgctgggtctctgggtaggagagccatttatctaataattcttctgaaagctttaggaggagggcaaagttactcttcagagaatcagtcacaccattttcatacaattttttcctcatgtggttttcactcacactgccaccaccagattgataccttaataatgacttcagcatggtttcaaaagggtccgctgctcggaaaagaacatttaagaaggtgtatggtcaattccagcagttcagctacttttcaactttcactgtaaaaccaccaccttgctttgtagaacaggtgttttttgtttgtttgtttgtttgttttgagataagagtctggctctgtcgccaggctgcagtgcagtggtgcgatcttggctcactgcaagctccgcctcccaggttcaagcgattctcctgcctcagcctcctgagtagctgggattacaggcgcccgccaccacagccagctaatgtttgtatttttagtagagacggtgtgtcaccatgttggccaggatggtctcgatatcctgacctcgtgatccgcccgcctcagcctcccaaagtgtgtagaacaggttttaaagacggtcctcagtcatcaacacttttgttttcagaccctccctctctcgctgacggaggcaagtggagagaggaggaccggaggctcgcagaggcgtcagcggcagaggaaacctcgcacccgaacccgcagcgcggcgctctccccaaagaagcatttgcctggagcccctaagaggagcaagacctggacctcgagcactttggattccagtcaggatagatcgatggacagatggaaaagaggaatacacaagtgctgggagaatcctcaagaaaggagaaaggagtggcgcgcccaggagtctcgtcctgacacactgggaaatgaaatttgggtttggcgagttatggccaaaaagctgcccaaagtacttgagagccgccttggagagtggcgcggggtgcctggcaaggtgagaccggcctgcgggggcgcgggcttttcctcagcagctctacgcccgcctggcccggcgcctgaggggtagc

SEQ ID NO: 15913 - RNA, 3986 nt, Homo sapiens
  source 1..3986: mol_type = other RNA
gctgggattacaggcatgagccatcacgcccggccaaagttttagaatttaagttattccaaaaaaaattttttttttcaaaaatacagactgcatccaattaaattctatgttaactggtaatgactaggtctaaaatgttaggtatttaccaataaatgacataaaataactcaacaacaaagggatttttttttttaagagatagggtctcactttatcactcaggtttggctgagggcagtggtgtgatcacagctcactgaagcctccaactcctgggctcaagtgatcctcccgcctcagtctaccagagtatattcttgaaagtaaaattacaaatgaaattcagcagtgttaaaaataagcccacttgcagacaattatcatttttcttcctttctttcctcactatctgtacttggcatatttcctacagtggctgtcttaaagaaaaaaaggaatccttcacaaatagtgtagccaaaaaagttggactaatatacaatgctatcagtaaagtattatatataaaatttataagtgctaaagtgtaattttgaaagacacttaagatactccttttttttttgagacaaggtctcagccctgtcgcccaggctggagtgcactagcacaacatcagctcactgcaacctccgcctcccaggttcaagcgattctcctgcctcagcctcccaagtagctgagactacaggcgcacgccagcatgtccagataattttttgtatttttagtagagatggggtttcaccatgttggccaggatggtctcaaatctcttgacctcgtgatctgcccatgtcggcttcccaaagtgttaggataacaggcatgagctaccgtgcccagcctacttaaaatattcttgaaatagctctccccacctccttttttttttttttttgagaatgagtttcactcgacacccaggctggagtgcagtggtgcgatcttggctcactgcaacctctgcctcccaggttcaagcgattatcctgcctcagcctcctgagtagctgggattacaaatgtgcaccaccacatctggctaattttttttttttttttttgtatttttagtagagacggggtttcaccaagttggcctggctggtctcgaacacctgacctcaattgatccacctgcctcggcctcccaaagtattataggcatgagccaccgagcccggccttttttgttttttgtttttttaaaggcagggttttgctctgttgcccaggctggagtgcagtggtgtgatcacagatcactgcagccttgacctctcctggtctcaagtgatcctcccacctcagccttcagaacagctgggactacaggtgtgtgtcaccatgcccagtaatttttttgtatatttgtagaggcagggtctcccaatgttgcctgggctggtctcaaactcctgggctcaagcaatccaccagctttggccttccaaagttctaggattatacgcatgagccactgtgccctgccccaatattttgttacttactagtgagactaaacacttttctaaaagtttgttagccatactatcctataaaagctgtttgttcatgtcttttgtccatttatctttttttttgtttttcttgagacagagtcttgctctgtggcccaggctggagtgcaggggtgcaatctcggctcactgcaagctccgcctcccaggttcaaatgattctcctgcctcagcctcctgagtagctgggattacaggcatgtgccaccatgcccagctaatttttttgtgtgtgtttttcagtagagatggggtttcaccatgttggccaggctgatctcgaattcctgacctcaggtgctccacccgcctcagcctcccaaagtactgggattacaggggtgagccaccgcacccggccaattttctgtatttttaatagagacagggtttcatcctgttggccaggctggcctcgaacttcggacctcaggtgatccacccgcctcgacctcccaaagtgctgggattacaggtgtgggccaccacacccagccaatttttttgtatttttagtagagacagggtttcatcatgttggccaggctggtcgcaaactcctgacctcaggtgatccacccgcctcagcatcccaaagtgctgggattacaggcatgagccaccactcccggccaatgttttgtatttttagtagagatggggtttcatcatgttggccagactggtctcaaactctggacctcaggtgatccacctgcctcagcctcccaaagtgtagggattacaggtgtgagccaccgcgcccagcctatgtttctattttatacatattcaacaaacatgattccccaacttctgcaaaataatttctttttcaagaacattgattttagagctcacactaagaaaaagaatacaaaaataatggcatagaaagtgaaaaaacaaaaataaaaagtagaaagctaaagtttcccattaaaatgatcaatatactgtgcagtaagtcaaatgtgtacaatgaattaagaaaatatgatatataaaaatccaaatttacaaaattaagtacaaataggtgtttatattacaaagtgatactggtttataaaaggattcaacatagattttttttaaatggttgttttcctcaatcaatttaacaatgattttaaatgtataaaattttaatatctctttgagacagtgatccaagcttcttcccttgatgatgttaccagttcatactttgtttcaataacctgtccctccacagaaagtaggtgcagtctcttcaccaatacactaagaagtactgtggtcaccatatatgcaaacctcaactctggacactcctgtgtgcctgagaatccaagtgaggaaaaagttttcattactaattcatcatcaaaccgatctggatcaaacttgtgtggagatggccaagtattaggatcctgaagtaccacaccaagggcataaaggacgagggtctctctaggaataataaatcggtcaatttttccttcaatatcttgaagctgggcagaaactggagtcagtttggcagttcgaacagtttcacaaagcacatgctgacaatatctgagctgctcaattttctctggagtaacaggaccatttccaaaaacttggtttatctcttcatataattttttttgaacttcttcagaggtggttaaaaaacagattgcccaggtacacaattttgcagttattatgcaactggccagagaaaatatcatactgtcttctaggatctgttggtcattaaggttcccttgtactaaggagtcaatgaaaatatgttgactgaagttccttccttttcgttcttttatgatgttccttaaaacagactccagttgcatgagggcatcttcatattgttttttccgagtcatgtttttatcaagtgacccatctagaaagccttttccaatctcagaccaaactgtgccatgattcttctggaagcgaatgacttcctgatcatcttcaaatgtactacccattaccatctgtgtaacagacttcatagcaaaaccaagcatatgctggctgaggggcacgtgctgggtctctgggtaggagagccatttatctaataattcttctgaaagctttaggaggagggcaaagttactcttcagagaatcagtcacaccattttcatacaattttttcctcatgtggttttcactcacactgccaccaccagattgataccttaataatgacttcagcatggtttcaaaagggtccgttttcttcagttggagtaatccctggaattcctgcagcttgtctggaagccggatagaggtagagcacggctcccaccaacgccagcaagaaggtaacggcgaagatcgcgaagtccaacatggttctgccgcccagggagccacgtctcggatcggccgctccagc

SEQ ID NO: 15914 - RNA, 3801 nt, Homo sapiens
  source 1..3801: mol_type = other RNA
gctgggattacaggcatgagccatcacgcccggccaaagttttagaatttaagttattccaaaaaaaattttttttttcaaaaatacagactgcatccaattaaattctatgttaactggtaatgactaggtctaaaatgttaggtatttaccaataaatgacataaaataactcaacaacaaagggatttttttttttaagagatagggtctcactttatcactcaggtttggctgagggcagtggtgtgatcacagctcactgaagcctccaactcctgggctcaagtgatcctcccgcctcagtctaccagagtatattcttgaaagtaaaattacaaatgaaattcagcagtgttaaaaataagcccacttgcagacaattatcatttttcttcctttctttcctcactatctgtacttggcatatttcctacagtggctgtcttaaagaaaaaaaggaatccttcacaaatagtgtagccaaaaaagttggactaatatacaatgctatcagtaaagtattatatataaaatttataagtgctaaagtgtaattttgaaagacacttaagatactccttttttttttgagacaaggtctcagccctgtcgcccaggctggagtgcactagcacaacatcagctcactgcaacctccgcctcccaggttcaagcgattctcctgcctcagcctcccaagtagctgagactacaggcgcacgccagcatgtccagataattttttgtatttttagtagagatggggtttcaccatgttggccaggatggtctcaaatctcttgacctcgtgatctgcccatgtcggcttcccaaagtgttaggataacaggcatgagctaccgtgcccagcctacttaaaatattcttgaaatagctctccccacctccttttttttttttttttgagaatgagtttcactcgacacccaggctggagtgcagtggtgcgatcttggctcactgcaacctctgcctcccaggttcaagcgattatcctgcctcagcctcctgagtagctgggattacaaatgtgcaccaccacatctggctaattttttttttttttttttgtatttttagtagagacggggtttcaccaagttggcctggctggtctcgaacacctgacctcaattgatccacctgcctcggcctcccaaagtattataggcatgagccaccgagcccggccttttttgttttttgtttttttaaaggcagggttttgctctgttgcccaggctggagtgcagtggtgtgatcacagatcactgcagccttgacctctcctggtctcaagtgatcctcccacctcagccttcagaacagctgggactacaggtgtgtgtcaccatgcccagtaatttttttgtatatttgtagaggcagggtctcccaatgttgcctgggctggtctcaaactcctgggctcaagcaatccaccagctttggccttccaaagttctaggattatacgcatgagccactgtgccctgccccaatattttgttacttactagtgagactaaacacttttctaaaagtttgttagccatactatcctataaaagctgtttgttcatgtcttttgtccatttatctttttttttgtttttcttgagacagagtcttgctctgtggcccaggctggagtgcaggggtgcaatctcggctcactgcaagctccgcctcccaggttcaaatgattctcctgcctcagcctcctgagtagctgggattacaggcatgtgccaccatgcccagctaatttttttgtgtgtgtttttcagtagagatggggtttcaccatgttggccaggctgatctcgaattcctgacctcaggtgctccacccgcctcagcctcccaaagtactgggattacaggggtgagccaccgcacccggccaattttctgtatttttaatagagacagggtttcatcctgttggccaggctggcctcgaacttcggacctcaggtgatccacccgcctcgacctcccaaagtgctgggattacaggtgtgggccaccacacccagccaatttttttgtatttttagtagagacagggtttcatcatgttggccaggctggtcgcaaactcctgacctcaggtgatccacccgcctcagcatcccaaagtgctgggattacaggcatgagccaccactcccggccaatgttttgtatttttagtagagatggggtttcatcatgttggccagactggtctcaaactctggacctcaggtgatccacctgcctcagcctcccaaagtgtagggattacaggtgtgagccaccgcgcccagcctatgtttctattttatacatattcaacaaacatgattccccaacttctgcaaaataatttctttttcaagaacattgattttagagctcacactaagaaaaagaatacaaaaataatggcatagaaagtgaaaaaacaaaaataaaaagtagaaagctaaagtttcccattaaaatgatcaatatactgtgcagtaagtcaaatgtgtacaatgaattaagaaaatatgatatataaaaatccaaatttacaaaattaagtacaaataggtgtttatattacaaagtgatactggtttataaaaggattcaacatagattttttttaaatggttgttttcctcaatcaatttaacaatgattttaaatgtataaaattttaatatctctttgagacagtgatccaagcttcttcccttgatgatgttaccagttcatactttgtttcaataacctgtccctccacagaaagtaggtgcagtctcttcaccaatacactaagaagtactgtggtcaccatatatgcaaacctcaactctggacactcctgtgtgcctgagaatccaagtgaggaaaaagttttcattactaattcatcatcaaaccgatctggatcaaacttgtgtggagatggccaagtattaggatcctgaagtaccacaccaagggcataaaggacgagggtctctctaggaataataaatcggtcaatttttccttcaatatcttgaagctgggcagaaactggagtcagtttggcagttcgaacagtttcacaaagcacatgctgacaatatctgagctgctcaattttctctggagtaacaggaccatttccaaaaacttggtttatctcttcatataattttttttgaacttcttcagaggtggttaaaaaacagattgcccaggtacacaattttgcagttattatgcaactggccagagaaaatatcatactgtcttctaggatctgttggtcattaaggttcccttgtactaaggagtcaatgaaaatatgttgactgaagttccttccttttcgttcttttatgatgttccttaaaacagactccagttgcatgagggtgtgccatgattcttctggaagcgaatgacttcctgatcatcttcaaatgtactacccattaccatctgtgtaacagacttcatagcaaaaccaagcatatgctggctgaggggcacgtgctgggtctctgggtaggagagccatttatctaataattcttctgaaagcttaataatgacttcagcatggtttcaaaagggtccgttttcttcagttggagtaatccctggaattcctgcagcttgtctggaagccggatagaggtagagcacggctcccaccaacgccagcaagaaggtaacggcgaagatcgcgaagtccaacatggttctgccgcccagggagccacgtctcggatcggccgctccagc

SEQ ID NO: 15915 - RNA, 4074 nt, Homo sapiens
  source 1..4074: mol_type = other RNA
gctgggattacaggcatgagccatcacgcccggccaaagttttagaatttaagttattccaaaaaaaattttttttttcaaaaatacagactgcatccaattaaattctatgttaactggtaatgactaggtctaaaatgttaggtatttaccaataaatgacataaaataactcaacaacaaagggatttttttttttaagagatagggtctcactttatcactcaggtttggctgagggcagtggtgtgatcacagctcactgaagcctccaactcctgggctcaagtgatcctcccgcctcagtctaccagagtatattcttgaaagtaaaattacaaatgaaattcagcagtgttaaaaataagcccacttgcagacaattatcatttttcttcctttctttcctcactatctgtacttggcatatttcctacagtggctgtcttaaagaaaaaaaggaatccttcacaaatagtgtagccaaaaaagttggactaatatacaatgctatcagtaaagtattatatataaaatttataagtgctaaagtgtaattttgaaagacacttaagatactccttttttttttgagacaaggtctcagccctgtcgcccaggctggagtgcactagcacaacatcagctcactgcaacctccgcctcccaggttcaagcgattctcctgcctcagcctcccaagtagctgagactacaggcgcacgccagcatgtccagataattttttgtatttttagtagagatggggtttcaccatgttggccaggatggtctcaaatctcttgacctcgtgatctgcccatgtcggcttcccaaagtgttaggataacaggcatgagctaccgtgcccagcctacttaaaatattcttgaaatagctctccccacctccttttttttttttttttgagaatgagtttcactcgacacccaggctggagtgcagtggtgcgatcttggctcactgcaacctctgcctcccaggttcaagcgattatcctgcctcagcctcctgagtagctgggattacaaatgtgcaccaccacatctggctaattttttttttttttttttgtatttttagtagagacggggtttcaccaagttggcctggctggtctcgaacacctgacctcaattgatccacctgcctcggcctcccaaagtattataggcatgagccaccgagcccggccttttttgttttttgtttttttaaaggcagggttttgctctgttgcccaggctggagtgcagtggtgtgatcacagatcactgcagccttgacctctcctggtctcaagtgatcctcccacctcagccttcagaacagctgggactacaggtgtgtgtcaccatgcccagtaatttttttgtatatttgtagaggcagggtctcccaatgttgcctgggctggtctcaaactcctgggctcaagcaatccaccagctttggccttccaaagttctaggattatacgcatgagccactgtgccctgccccaatattttgttacttactagtgagactaaacacttttctaaaagtttgttagccatactatcctataaaagctgtttgttcatgtcttttgtccatttatctttttttttgtttttcttgagacagagtcttgctctgtggcccaggctggagtgcaggggtgcaatctcggctcactgcaagctccgcctcccaggttcaaatgattctcctgcctcagcctcctgagtagctgggattacaggcatgtgccaccatgcccagctaatttttttgtgtgtgtttttcagtagagatggggtttcaccatgttggccaggctgatctcgaattcctgacctcaggtgctccacccgcctcagcctcccaaagtactgggattacaggggtgagccaccgcacccggccaattttctgtatttttaatagagacagggtttcatcctgttggccaggctggcctcgaacttcggacctcaggtgatccacccgcctcgacctcccaaagtgctgggattacaggtgtgggccaccacacccagccaatttttttgtatttttagtagagacagggtttcatcatgttggccaggctggtcgcaaactcctgacctcaggtgatccacccgcctcagcatcccaaagtgctgggattacaggcatgagccaccactcccggccaatgttttgtatttttagtagagatggggtttcatcatgttggccagactggtctcaaactctggacctcaggtgatccacctgcctcagcctcccaaagtgtagggattacaggtgtgagccaccgcgcccagcctatgtttctattttatacatattcaacaaacatgattccccaacttctgcaaaataatttctttttcaagaacattgattttagagctcacactaagaaaaagaatacaaaaataatggcatagaaagtgaaaaaacaaaaataaaaagtagaaagctaaagtttcccattaaaatgatcaatatactgtgcagtaagtcaaatgtgtacaatgaattaagaaaatatgatatataaaaatccaaatttacaaaattaagtacaaataggtgtttatattacaaagtgatactggtttataaaaggattcaacatagattttttttaaatggttgttttcctcaatcaatttaacaatgattttaaatgtataaaattttaatatctctttgagacagtgatccaagcttcttcccttgatgatgttaccagttcatactttgtttcaataacctgtccctccacagaaagtaggtgcagtctcttcaccaatacactaagaagtactgtggtcaccatatatgcaaacctcaactctggacactcctgtgtgcctgagaatccaagtgaggaaaaagttttcattactaattcatcatcaaaccgatctggatcaaacttgtgtggagatggccaagtattaggatcctgaagtaccacaccaagggcataaaggacgagggtctctctaggaataataaatcggtcaatttttccttcaatatcttgaagctgggcagaaactggagtcagtttggcagttcgaacagtttcacaaagcacatgctgacaatatctgagctgctcaattttctctggagtaacaggaccatttccaaaaacttggtttatctcttcatataattttttttgaacttcttcagaggtggttaaaaaacagattgcccaggtacacaattttgcagttattatgcaactggccagagaaaatatcatactgtcttctaggatctgttggtcattaaggttcccttgtactaaggagtcaatgaaaatatgttgactgaagttccttccttttcgttcttttatgatgttccttaaaacagactccagttgcatgagggtgtgccatgattcttctggaagcgaatgacttcctgatcatcttcaaatgtactacccattaccatctgtgtaacagacttcatagcaaaaccaagcatatgctggctgaggggcacgtgctgggtctctgggtaggagagccatttatctaataattcttctgaaagctttaggaggagggcaaagttactcttcagagaatcagtcacaccattttcatacaattttttcctcatgtggttttcactcacactgccaccaccagattgataccttaataatgacttcagcatggtttcaaaagggtccgatgtcttattgggattgatatgctgcttcagtacatcaacagtgcccaaactaaccacgaggcgcctgccaaaccagaaggagaccacaggcccatatctctcatgcaaattaaccaggaactcatgcaaacttccactattcacaatatctggaagattaccatctttttcttcagttggagtaatccctggaattcctgcagcttgtctggaagccggatagaggtagagcacggctcccaccaacgccagcaagaaggtaacggcgaagatcgcgaagtccaacatggttctgccgcccagggagccacgtctcggatcggccgctccagc

SEQ ID NO: 15916 - RNA, 3857 nt, Homo sapiens
  source 1..3857: mol_type = other RNA
gctgggattacaggcatgagccatcacgcccggccaaagttttagaatttaagttattccaaaaaaaattttttttttcaaaaatacagactgcatccaattaaattctatgttaactggtaatgactaggtctaaaatgttaggtatttaccaataaatgacataaaataactcaacaacaaagggatttttttttttaagagatagggtctcactttatcactcaggtttggctgagggcagtggtgtgatcacagctcactgaagcctccaactcctgggctcaagtgatcctcccgcctcagtctaccagagtatattcttgaaagtaaaattacaaatgaaattcagcagtgttaaaaataagcccacttgcagacaattatcatttttcttcctttctttcctcactatctgtacttggcatatttcctacagtggctgtcttaaagaaaaaaaggaatccttcacaaatagtgtagccaaaaaagttggactaatatacaatgctatcagtaaagtattatatataaaatttataagtgctaaagtgtaattttgaaagacacttaagatactccttttttttttgagacaaggtctcagccctgtcgcccaggctggagtgcactagcacaacatcagctcactgcaacctccgcctcccaggttcaagcgattctcctgcctcagcctcccaagtagctgagactacaggcgcacgccagcatgtccagataattttttgtatttttagtagagatggggtttcaccatgttggccaggatggtctcaaatctcttgacctcgtgatctgcccatgtcggcttcccaaagtgttaggataacaggcatgagctaccgtgcccagcctacttaaaatattcttgaaatagctctccccacctccttttttttttttttttgagaatgagtttcactcgacacccaggctggagtgcagtggtgcgatcttggctcactgcaacctctgcctcccaggttcaagcgattatcctgcctcagcctcctgagtagctgggattacaaatgtgcaccaccacatctggctaattttttttttttttttttgtatttttagtagagacggggtttcaccaagttggcctggctggtctcgaacacctgacctcaattgatccacctgcctcggcctcccaaagtattataggcatgagccaccgagcccggccttttttgttttttgtttttttaaaggcagggttttgctctgttgcccaggctggagtgcagtggtgtgatcacagatcactgcagccttgacctctcctggtctcaagtgatcctcccacctcagccttcagaacagctgggactacaggtgtgtgtcaccatgcccagtaatttttttgtatatttgtagaggcagggtctcccaatgttgcctgggctggtctcaaactcctgggctcaagcaatccaccagctttggccttccaaagttctaggattatacgcatgagccactgtgccctgccccaatattttgttacttactagtgagactaaacacttttctaaaagtttgttagccatactatcctataaaagctgtttgttcatgtcttttgtccatttatctttttttttgtttttcttgagacagagtcttgctctgtggcccaggctggagtgcaggggtgcaatctcggctcactgcaagctccgcctcccaggttcaaatgattctcctgcctcagcctcctgagtagctgggattacaggcatgtgccaccatgcccagctaatttttttgtgtgtgtttttcagtagagatggggtttcaccatgttggccaggctgatctcgaattcctgacctcaggtgctccacccgcctcagcctcccaaagtactgggattacaggggtgagccaccgcacccggccaattttctgtatttttaatagagacagggtttcatcctgttggccaggctggcctcgaacttcggacctcaggtgatccacccgcctcgacctcccaaagtgctgggattacaggtgtgggccaccacacccagccaatttttttgtatttttagtagagacagggtttcatcatgttggccaggctggtcgcaaactcctgacctcaggtgatccacccgcctcagcatcccaaagtgctgggattacaggcatgagccaccactcccggccaatgttttgtatttttagtagagatggggtttcatcatgttggccagactggtctcaaactctggacctcaggtgatccacctgcctcagcctcccaaagtgtagggattacaggtgtgagccaccgcgcccagcctatgtttctattttatacatattcaacaaacatgattccccaacttctgcaaaataatttctttttcaagaacattgattttagagctcacactaagaaaaagaatacaaaaataatggcatagaaagtgaaaaaacaaaaataaaaagtagaaagctaaagtttcccattaaaatgatcaatatactgtgcagtaagtcaaatgtgtacaatgaattaagaaaatatgatatataaaaatccaaatttacaaaattaagtacaaataggtgtttatattacaaagtgatactggtttataaaaggattcaacatagattttttttaaatggttgttttcctcaatcaatttaacaatgattttaaatgtataaaattttaatatctctttgagacagtgatccaagcttcttcccttgatgatgttaccagttcatactttgtttcaataacctgtccctccacagaaagtaggtgcagtctcttcaccaatacactaagaagtactgtggtcaccatatatgcaaacctcaactctggacactcctgtgtgcctgagaatccaagtgaggaaaaagttttcattactaattcatcatcaaaccgatctggatcaaacttgtgtggagatggccaagtattaggatcctgaagtaccacaccaagggcataaaggacgagggtctctctaggaataataaatcggtcaatttttccttcaatatcttgaagctgggcagaaactggagtcagtttggcagttcgaacagtttcacaaagcacatgctgacaatatctgagctgctcaattttctctggagtaacaggaccatttccaaaaacttggtttatctcttcatataattttttttgaacttcttcagaggtggttaaaaaacagattgcccaggtacacaattttgcagttattatgcaactggccagagaaaatatcatactgtcttctaggatctgttggtcattaaggttcccttgtactaaggagtcaatgaaaatatgttgactgaagttccttccttttcgttcttttatgatgttccttaaaacagactccagttgcatgagggtgtgccatgattcttctggaagcgaatgacttcctgatcatcttcaaatgtactacccattaccatctgtgtaacagacttcatagcaaaaccaagcatatgctggctgaggggcacgtgctgggtctctgggtaggagagccatttatctaataattcttctgaaagctttaggaggagggcaaagttactcttcagagaatcagtcacaccattttcatacaattttttcctcatgtggttttcactcacactgccaccaccagattgataccttaataatgacttcagcatggtttcaaaagggtccgcggatagaggtagagcacggctcccaccaacgccagcaagaaggtaacggcgaagatcgcgaagtccaacatggttctgccgcccagggagccacgtctcggatcggccgctccagc

SEQ ID NO: 15917 - RNA, 4626 nt, Homo sapiens
  source 1..4626: mol_type = other RNA
gctgggattacaggcatgagccatcacgcccggccaaagttttagaatttaagttattccaaaaaaaattttttttttcaaaaatacagactgcatccaattaaattctatgttaactggtaatgactaggtctaaaatgttaggtatttaccaataaatgacataaaataactcaacaacaaagggatttttttttttaagagatagggtctcactttatcactcaggtttggctgagggcagtggtgtgatcacagctcactgaagcctccaactcctgggctcaagtgatcctcccgcctcagtctaccagagtatattcttgaaagtaaaattacaaatgaaattcagcagtgttaaaaataagcccacttgcagacaattatcatttttcttcctttctttcctcactatctgtacttggcatatttcctacagtggctgtcttaaagaaaaaaaggaatccttcacaaatagtgtagccaaaaaagttggactaatatacaatgctatcagtaaagtattatatataaaatttataagtgctaaagtgtaattttgaaagacacttaagatactccttttttttttgagacaaggtctcagccctgtcgcccaggctggagtgcactagcacaacatcagctcactgcaacctccgcctcccaggttcaagcgattctcctgcctcagcctcccaagtagctgagactacaggcgcacgccagcatgtccagataattttttgtatttttagtagagatggggtttcaccatgttggccaggatggtctcaaatctcttgacctcgtgatctgcccatgtcggcttcccaaagtgttaggataacaggcatgagctaccgtgcccagcctacttaaaatattcttgaaatagctctccccacctccttttttttttttttttgagaatgagtttcactcgacacccaggctggagtgcagtggtgcgatcttggctcactgcaacctctgcctcccaggttcaagcgattatcctgcctcagcctcctgagtagctgggattacaaatgtgcaccaccacatctggctaattttttttttttttttttgtatttttagtagagacggggtttcaccaagttggcctggctggtctcgaacacctgacctcaattgatccacctgcctcggcctcccaaagtattataggcatgagccaccgagcccggccttttttgttttttgtttttttaaaggcagggttttgctctgttgcccaggctggagtgcagtggtgtgatcacagatcactgcagccttgacctctcctggtctcaagtgatcctcccacctcagccttcagaacagctgggactacaggtgtgtgtcaccatgcccagtaatttttttgtatatttgtagaggcagggtctcccaatgttgcctgggctggtctcaaactcctgggctcaagcaatccaccagctttggccttccaaagttctaggattatacgcatgagccactgtgccctgccccaatattttgttacttactagtgagactaaacacttttctaaaagtttgttagccatactatcctataaaagctgtttgttcatgtcttttgtccatttatctttttttttgtttttcttgagacagagtcttgctctgtggcccaggctggagtgcaggggtgcaatctcggctcactgcaagctccgcctcccaggttcaaatgattctcctgcctcagcctcctgagtagctgggattacaggcatgtgccaccatgcccagctaatttttttgtgtgtgtttttcagtagagatggggtttcaccatgttggccaggctgatctcgaattcctgacctcaggtgctccacccgcctcagcctcccaaagtactgggattacaggggtgagccaccgcacccggccaattttctgtatttttaatagagacagggtttcatcctgttggccaggctggcctcgaacttcggacctcaggtgatccacccgcctcgacctcccaaagtgctgggattacaggtgtgggccaccacacccagccaatttttttgtatttttagtagagacagggtttcatcatgttggccaggctggtcgcaaactcctgacctcaggtgatccacccgcctcagcatcccaaagtgctgggattacaggcatgagccaccactcccggccaatgttttgtatttttagtagagatggggtttcatcatgttggccagactggtctcaaactctggacctcaggtgatccacctgcctcagcctcccaaagtgtagggattacaggtgtgagccaccgcgcccagcctatgtttctattttatacatattcaacaaacatgattccccaacttctgcaaaataatttctttttcaagaacattgattttagagctcacactaagaaaaagaatacaaaaataatggcatagaaagtgaaaaaacaaaaataaaaagtagaaagctaaagtttcccattaaaatgatcaatatactgtgcagtaagtcaaatgtgtacaatgaattaagaaaatatgatatataaaaatccaaatttacaaaattaagtacaaataggtgtttatattacaaagtgatactggtttataaaaggattcaacatagattttttttaaatggttgttttcctcaatcaatttaacaatgattttaaatgtataaaattttaatatctctttgagacagtgatccaagcttcttcccttgatgatgttaccagttcatactttgtttcaataacctgtccctccacagaaagtaggtgcagtctcttcaccaatacactaagaagtactgtggtcaccatatatgcaaacctcaactctggacactcctgtgtgcctgagaatccaagtgaggaaaaagttttcattactaattcatcatcaaaccgatctggatcaaacttgtgtggagatggccaagtattaggatcctgaagtaccacaccaagggcataaaggacgagggtctctctaggaataataaatcggtcaatttttccttcaatatcttgaagctgggcagaaactggagtcagtttggcagttcgaacagtttcacaaagcacatgctgacaatatctgagctgctcaattttctctggagtaacaggaccatttccaaaaacttggtttatctcttcatataattttttttgaacttcttcagaggtggttaaaaaacagattgcccaggtacacaattttgcagttattatgcaactggccagagaaaatatcatactgtcttctaggatctgttggtcattaaggttcccttgtactaaggagtcaatgaaaatatgttgactgaagttccttccttttcgttcttttatgatgttccttaaaacagactccagttgcatgagggtgtgccatgattcttctggaagcgaatgacttcctgatcatcttcaaatgtactacccattaccatctgtgtaacagacttcatagcaaaaccaagcatatgctggctgaggggcacgtgctgggtctctgggtaggagagccatttatctaataattcttctgaaagctttaggaggagggcaaagttactcttcagagaatcagtcacaccattttcatacaattttttcctcatgtggttttcactcacactgccaccaccagattgataccttaataatgacttcagcatggtttcaaaagggtccgctgctcggaaaagaacatttaagaaggtgtatggtcaattccagcagttcagctacttttcaactttcactgtaaaaccaccaccttgctttgtagaacaggtgttttttgtttgtttgtttgtttgttttgagataagagtctggctctgtcgccaggctgcagtgcagtggtgcgatcttggctcactgcaagctccgcctcccaggttcaagcgattctcctgcctcagcctcctgagtagctgggattacaggcgcccgccaccacagccagctaatgtttgtatttttagtagagacggtgtgtcaccatgttggccaggatggtctcgatatcctgacctcgtgatccgcccgcctcagcctcccaaagtgtgtagaacaggttttaaagacggtcctcagtcatcaacacttttgttttcagaccctccctctctcgctgacggaggcaagtggagagaggaggaccggaggctcgcagaggcgtcagcggcagaggaaacctcgcacccgaacccgcagcgcggcgctctccccaaagaagcatttgcctggagcccctaagaggagcaagacctggacctcgagcactttggattccagtcaggatagatcgatggacagatggaaaagaggaatacacaagtgctgggagaatcctcaagaaaggagaaaggagtggcgcgcccaggagtctcgtcctgacacactgggaaatgaaatttgggtttggcgagttatggccaaaaagctgcccaaagtacttgagagccgccttggagagtggcgcggggtgcctggcaaggtgagaccggcctgcgggggcgcgggcttttcctcagcagctctacgcccgcctggcccggcgcctgaggggtagc

SEQ ID NO: 15918 - RNA, 3907 nt, Homo sapiens
  source 1..3907: mol_type = other RNA
gctgggattacaggcatgagccatcacgcccggccaaagttttagaatttaagttattccaaaaaaaattttttttttcaaaaatacagactgcatccaattaaattctatgttaactggtaatgactaggtctaaaatgttaggtatttaccaataaatgacataaaataactcaacaacaaagggatttttttttttaagagatagggtctcactttatcactcaggtttggctgagggcagtggtgtgatcacagctcactgaagcctccaactcctgggctcaagtgatcctcccgcctcagtctaccagagtatattcttgaaagtaaaattacaaatgaaattcagcagtgttaaaaataagcccacttgcagacaattatcatttttcttcctttctttcctcactatctgtacttggcatatttcctacagtggctgtcttaaagaaaaaaaggaatccttcacaaatagtgtagccaaaaaagttggactaatatacaatgctatcagtaaagtattatatataaaatttataagtgctaaagtgtaattttgaaagacacttaagatactccttttttttttgagacaaggtctcagccctgtcgcccaggctggagtgcactagcacaacatcagctcactgcaacctccgcctcccaggttcaagcgattctcctgcctcagcctcccaagtagctgagactacaggcgcacgccagcatgtccagataattttttgtatttttagtagagatggggtttcaccatgttggccaggatggtctcaaatctcttgacctcgtgatctgcccatgtcggcttcccaaagtgttaggataacaggcatgagctaccgtgcccagcctacttaaaatattcttgaaatagctctccccacctccttttttttttttttttgagaatgagtttcactcgacacccaggctggagtgcagtggtgcgatcttggctcactgcaacctctgcctcccaggttcaagcgattatcctgcctcagcctcctgagtagctgggattacaaatgtgcaccaccacatctggctaattttttttttttttttttgtatttttagtagagacggggtttcaccaagttggcctggctggtctcgaacacctgacctcaattgatccacctgcctcggcctcccaaagtattataggcatgagccaccgagcccggccttttttgttttttgtttttttaaaggcagggttttgctctgttgcccaggctggagtgcagtggtgtgatcacagatcactgcagccttgacctctcctggtctcaagtgatcctcccacctcagccttcagaacagctgggactacaggtgtgtgtcaccatgcccagtaatttttttgtatatttgtagaggcagggtctcccaatgttgcctgggctggtctcaaactcctgggctcaagcaatccaccagctttggccttccaaagttctaggattatacgcatgagccactgtgccctgccccaatattttgttacttactagtgagactaaacacttttctaaaagtttgttagccatactatcctataaaagctgtttgttcatgtcttttgtccatttatctttttttttgtttttcttgagacagagtcttgctctgtggcccaggctggagtgcaggggtgcaatctcggctcactgcaagctccgcctcccaggttcaaatgattctcctgcctcagcctcctgagtagctgggattacaggcatgtgccaccatgcccagctaatttttttgtgtgtgtttttcagtagagatggggtttcaccatgttggccaggctgatctcgaattcctgacctcaggtgctccacccgcctcagcctcccaaagtactgggattacaggggtgagccaccgcacccggccaattttctgtatttttaatagagacagggtttcatcctgttggccaggctggcctcgaacttcggacctcaggtgatccacccgcctcgacctcccaaagtgctgggattacaggtgtgggccaccacacccagccaatttttttgtatttttagtagagacagggtttcatcatgttggccaggctggtcgcaaactcctgacctcaggtgatccacccgcctcagcatcccaaagtgctgggattacaggcatgagccaccactcccggccaatgttttgtatttttagtagagatggggtttcatcatgttggccagactggtctcaaactctggacctcaggtgatccacctgcctcagcctcccaaagtgtagggattacaggtgtgagccaccgcgcccagcctatgtttctattttatacatattcaacaaacatgattccccaacttctgcaaaataatttctttttcaagaacattgattttagagctcacactaagaaaaagaatacaaaaataatggcatagaaagtgaaaaaacaaaaataaaaagtagaaagctaaagtttcccattaaaatgatcaatatactgtgcagtaagtcaaatgtgtacaatgaattaagaaaatatgatatataaaaatccaaatttacaaaattaagtacaaataggtgtttatattacaaagtgatactggtttataaaaggattcaacatagattttttttaaatggttgttttcctcaatcaatttaacaatgattttaaatgtataaaattttaatatctctttgagacagtgatccaagcttcttcccttgatgatgttaccagttcatactttgtttcaataacctgtccctccacagaaagtaggtgcagtctcttcaccaatacactaagaagtactgtggtcaccatatatgcaaacctcaactctggacactcctgtgtgcctgagaatccaagtgaggaaaaagttttcattactaattcatcatcaaaccgatctggatcaaacttgtgtggagatggccaagtattaggatcctgaagtaccacaccaagggcataaaggacgagggtctctctaggaataataaatcggtcaatttttccttcaatatcttgaagctgggcagaaactggagtcagtttggcagttcgaacagtttcacaaagcacatgctgacaatatctgagctgctcaattttctctggagtaacaggaccatttccaaaaacttggtttatctcttcatataattttttttgaacttcttcagaggtggttaaaaaacagattgcccaggtacacaattttgcagttattatgcaactggccagagaaaatatcatactgtcttctaggatctgttggtcattaaggttcccttgtactaaggagtcaatgaaaatatgttgactgaagttccttccttttcgttcttttatgatgttccttaaaacagactccagttgcatgagggtgtgccatgattcttctggaagcgaatgacttcctgatcatcttcaaatgtactacccattaccatctgtgtaacagacttcatagcaaaaccaagcatatgctggctgaggggcacgtgctgggtctctgggtaggagagccatttatctaataattcttctgaaagctttaggaggagggcaaagttactcttcagagaatcagtcacaccattttcatacaattttttcctcatgtggttttcactcacactgccaccaccagattgataccttaataatgacttcagcatggtttcaaaagggtccgttttcttcagttggagtaatccctggaattcctgcagcttgtctggaagccggatagaggtagagcacggctcccaccaacgccagcaagaaggtaacggcgaagatcgcgaagtccaacatggttctgccgcccagggagccacgtctcggatcggccgctccagc

SEQ ID NO: 15919 - RNA, 3741 nt, Homo sapiens
  source 1..3741: mol_type = other RNA
gctgggattacaggcatgagccatcacgcccggccaaagttttagaatttaagttattccaaaaaaaattttttttttcaaaaatacagactgcatccaattaaattctatgttaactggtaatgactaggtctaaaatgttaggtatttaccaataaatgacataaaataactcaacaacaaagggatttttttttttaagagatagggtctcactttatcactcaggtttggctgagggcagtggtgtgatcacagctcactgaagcctccaactcctgggctcaagtgatcctcccgcctcagtctaccagagtatattcttgaaagtaaaattacaaatgaaattcagcagtgttaaaaataagcccacttgcagacaattatcatttttcttcctttctttcctcactatctgtacttggcatatttcctacagtggctgtcttaaagaaaaaaaggaatccttcacaaatagtgtagccaaaaaagttggactaatatacaatgctatcagtaaagtattatatataaaatttataagtgctaaagtgtaattttgaaagacacttaagatactccttttttttttgagacaaggtctcagccctgtcgcccaggctggagtgcactagcacaacatcagctcactgcaacctccgcctcccaggttcaagcgattctcctgcctcagcctcccaagtagctgagactacaggcgcacgccagcatgtccagataattttttgtatttttagtagagatggggtttcaccatgttggccaggatggtctcaaatctcttgacctcgtgatctgcccatgtcggcttcccaaagtgttaggataacaggcatgagctaccgtgcccagcctacttaaaatattcttgaaatagctctccccacctccttttttttttttttttgagaatgagtttcactcgacacccaggctggagtgcagtggtgcgatcttggctcactgcaacctctgcctcccaggttcaagcgattatcctgcctcagcctcctgagtagctgggattacaaatgtgcaccaccacatctggctaattttttttttttttttttgtatttttagtagagacggggtttcaccaagttggcctggctggtctcgaacacctgacctcaattgatccacctgcctcggcctcccaaagtattataggcatgagccaccgagcccggccttttttgttttttgtttttttaaaggcagggttttgctctgttgcccaggctggagtgcagtggtgtgatcacagatcactgcagccttgacctctcctggtctcaagtgatcctcccacctcagccttcagaacagctgggactacaggtgtgtgtcaccatgcccagtaatttttttgtatatttgtagaggcagggtctcccaatgttgcctgggctggtctcaaactcctgggctcaagcaatccaccagctttggccttccaaagttctaggattatacgcatgagccactgtgccctgccccaatattttgttacttactagtgagactaaacacttttctaaaagtttgttagccatactatcctataaaagctgtttgttcatgtcttttgtccatttatctttttttttgtttttcttgagacagagtcttgctctgtggcccaggctggagtgcaggggtgcaatctcggctcactgcaagctccgcctcccaggttcaaatgattctcctgcctcagcctcctgagtagctgggattacaggcatgtgccaccatgcccagctaatttttttgtgtgtgtttttcagtagagatggggtttcaccatgttggccaggctgatctcgaattcctgacctcaggtgctccacccgcctcagcctcccaaagtactgggattacaggggtgagccaccgcacccggccaattttctgtatttttaatagagacagggtttcatcctgttggccaggctggcctcgaacttcggacctcaggtgatccacccgcctcgacctcccaaagtgctgggattacaggtgtgggccaccacacccagccaatttttttgtatttttagtagagacagggtttcatcatgttggccaggctggtcgcaaactcctgacctcaggtgatccacccgcctcagcatcccaaagtgctgggattacaggcatgagccaccactcccggccaatgttttgtatttttagtagagatggggtttcatcatgttggccagactggtctcaaactctggacctcaggtgatccacctgcctcagcctcccaaagtgtagggattacaggtgtgagccaccgcgcccagcctatgtttctattttatacatattcaacaaacatgattccccaacttctgcaaaataatttctttttcaagaacattgattttagagctcacactaagaaaaagaatacaaaaataatggcatagaaagtgaaaaaacaaaaataaaaagtagaaagctaaagtttcccattaaaatgatcaatatactgtgcagtaagtcaaatgtgtacaatgaattaagaaaatatgatatataaaaatccaaatttacaaaattaagtacaaataggtgtttatattacaaagtgatactggtttataaaaggattcaacatagattttttttaaatggttgttttcctcaatcaatttaacaatgattttaaatgtataaaattttaatatctctttgagacagtgatccaagcttcttcccttgatgatgttaccagttcatactttgtttcaataacctgtccctccacagaaagtaggtgcagtctcttcaccaatacactaagaagtactgtggtcaccatatatgcaaacctcaactctggacactcctgtgtgcctgagaatccaagtgaggaaaaagttttcattactaattcatcatcaaaccgatctggatcaaacttgtgtggagatggccaagtattaggatcctgaagtaccacaccaagggcataaaggacgagggtctctctaggaataataaatcggtcaatttttccttcaatatcttgaagctgggcagaaactggagtcagtttggcagttcgaacagtttcacaaagcacatgctgacaatatctgagctgctcaattttctctggagtaacaggaccatttccaaaaacttggtttatctcttcatataattttttttgaacttcttcagaggtggttaaaaaacagattgcccaggtacacaattttgcagttattatgcaactggccagagaaaatatcatactgtcttctaggattgtgccatgattcttctggaagcgaatgacttcctgatcatcttcaaatgtactacccattaccatctgtgtaacagacttcatagcaaaaccaagcatatgctggctgaggggcacgtgctgggtctctgggtaggagagccatttatctaataattcttctgaaagctttaggaggagggcaaagttactcttcagagaatcagtcacaccattttcatacaattttttcctcatgtggttttcactcacactgccaccaccagattgataccttaataatgacttcagcatggtttcaaaagggtccgcggatagaggtagagcacggctcccaccaacgccagcaagaaggtaacggcgaagatcgcgaagtccaacatggttctgccgcccagggagccacgtctcggatcggccgctccagc

SEQ ID NO: 15920 - RNA, 3791 nt, Homo sapiens
  source 1..3791: mol_type = other RNA
gctgggattacaggcatgagccatcacgcccggccaaagttttagaatttaagttattccaaaaaaaattttttttttcaaaaatacagactgcatccaattaaattctatgttaactggtaatgactaggtctaaaatgttaggtatttaccaataaatgacataaaataactcaacaacaaagggatttttttttttaagagatagggtctcactttatcactcaggtttggctgagggcagtggtgtgatcacagctcactgaagcctccaactcctgggctcaagtgatcctcccgcctcagtctaccagagtatattcttgaaagtaaaattacaaatgaaattcagcagtgttaaaaataagcccacttgcagacaattatcatttttcttcctttctttcctcactatctgtacttggcatatttcctacagtggctgtcttaaagaaaaaaaggaatccttcacaaatagtgtagccaaaaaagttggactaatatacaatgctatcagtaaagtattatatataaaatttataagtgctaaagtgtaattttgaaagacacttaagatactccttttttttttgagacaaggtctcagccctgtcgcccaggctggagtgcactagcacaacatcagctcactgcaacctccgcctcccaggttcaagcgattctcctgcctcagcctcccaagtagctgagactacaggcgcacgccagcatgtccagataattttttgtatttttagtagagatggggtttcaccatgttggccaggatggtctcaaatctcttgacctcgtgatctgcccatgtcggcttcccaaagtgttaggataacaggcatgagctaccgtgcccagcctacttaaaatattcttgaaatagctctccccacctccttttttttttttttttgagaatgagtttcactcgacacccaggctggagtgcagtggtgcgatcttggctcactgcaacctctgcctcccaggttcaagcgattatcctgcctcagcctcctgagtagctgggattacaaatgtgcaccaccacatctggctaattttttttttttttttttgtatttttagtagagacggggtttcaccaagttggcctggctggtctcgaacacctgacctcaattgatccacctgcctcggcctcccaaagtattataggcatgagccaccgagcccggccttttttgttttttgtttttttaaaggcagggttttgctctgttgcccaggctggagtgcagtggtgtgatcacagatcactgcagccttgacctctcctggtctcaagtgatcctcccacctcagccttcagaacagctgggactacaggtgtgtgtcaccatgcccagtaatttttttgtatatttgtagaggcagggtctcccaatgttgcctgggctggtctcaaactcctgggctcaagcaatccaccagctttggccttccaaagttctaggattatacgcatgagccactgtgccctgccccaatattttgttacttactagtgagactaaacacttttctaaaagtttgttagccatactatcctataaaagctgtttgttcatgtcttttgtccatttatctttttttttgtttttcttgagacagagtcttgctctgtggcccaggctggagtgcaggggtgcaatctcggctcactgcaagctccgcctcccaggttcaaatgattctcctgcctcagcctcctgagtagctgggattacaggcatgtgccaccatgcccagctaatttttttgtgtgtgtttttcagtagagatggggtttcaccatgttggccaggctgatctcgaattcctgacctcaggtgctccacccgcctcagcctcccaaagtactgggattacaggggtgagccaccgcacccggccaattttctgtatttttaatagagacagggtttcatcctgttggccaggctggcctcgaacttcggacctcaggtgatccacccgcctcgacctcccaaagtgctgggattacaggtgtgggccaccacacccagccaatttttttgtatttttagtagagacagggtttcatcatgttggccaggctggtcgcaaactcctgacctcaggtgatccacccgcctcagcatcccaaagtgctgggattacaggcatgagccaccactcccggccaatgttttgtatttttagtagagatggggtttcatcatgttggccagactggtctcaaactctggacctcaggtgatccacctgcctcagcctcccaaagtgtagggattacaggtgtgagccaccgcgcccagcctatgtttctattttatacatattcaacaaacatgattccccaacttctgcaaaataatttctttttcaagaacattgattttagagctcacactaagaaaaagaatacaaaaataatggcatagaaagtgaaaaaacaaaaataaaaagtagaaagctaaagtttcccattaaaatgatcaatatactgtgcagtaagtcaaatgtgtacaatgaattaagaaaatatgatatataaaaatccaaatttacaaaattaagtacaaataggtgtttatattacaaagtgatactggtttataaaaggattcaacatagattttttttaaatggttgttttcctcaatcaatttaacaatgattttaaatgtataaaattttaatatctctttgagacagtgatccaagcttcttcccttgatgatgttaccagttcatactttgtttcaataacctgtccctccacagaaagtaggtgcagtctcttcaccaatacactaagaagtactgtggtcaccatatatgcaaacctcaactctggacactcctgtgtgcctgagaatccaagtgaggaaaaagttttcattactaattcatcatcaaaccgatctggatcaaacttgtgtggagatggccaagtattaggatcctgaagtaccacaccaagggcataaaggacgagggtctctctaggaataataaatcggtcaatttttccttcaatatcttgaagctgggcagaaactggagtcagtttggcagttcgaacagtttcacaaagcacatgctgacaatatctgagctgctcaattttctctggagtaacaggaccatttccaaaaacttggtttatctcttcatataattttttttgaacttcttcagaggtggttaaaaaacagattgcccaggtacacaattttgcagttattatgcaactggccagagaaaatatcatactgtcttctaggattgtgccatgattcttctggaagcgaatgacttcctgatcatcttcaaatgtactacccattaccatctgtgtaacagacttcatagcaaaaccaagcatatgctggctgaggggcacgtgctgggtctctgggtaggagagccatttatctaataattcttctgaaagctttaggaggagggcaaagttactcttcagagaatcagtcacaccattttcatacaattttttcctcatgtggttttcactcacactgccaccaccagattgataccttaataatgacttcagcatggtttcaaaagggtccgttttcttcagttggagtaatccctggaattcctgcagcttgtctggaagccggatagaggtagagcacggctcccaccaacgccagcaagaaggtaacggcgaagatcgcgaagtccaacatggttctgccgcccagggagccacgtctcggatcggccgctccagc

SEQ ID NO: 15921 - RNA, 4041 nt, Homo sapiens
  source 1..4041: mol_type = other RNA
gctgggattacaggcatgagccatcacgcccggccaaagttttagaatttaagttattccaaaaaaaattttttttttcaaaaatacagactgcatccaattaaattctatgttaactggtaatgactaggtctaaaatgttaggtatttaccaataaatgacataaaataactcaacaacaaagggatttttttttttaagagatagggtctcactttatcactcaggtttggctgagggcagtggtgtgatcacagctcactgaagcctccaactcctgggctcaagtgatcctcccgcctcagtctaccagagtatattcttgaaagtaaaattacaaatgaaattcagcagtgttaaaaataagcccacttgcagacaattatcatttttcttcctttctttcctcactatctgtacttggcatatttcctacagtggctgtcttaaagaaaaaaaggaatccttcacaaatagtgtagccaaaaaagttggactaatatacaatgctatcagtaaagtattatatataaaatttataagtgctaaagtgtaattttgaaagacacttaagatactccttttttttttgagacaaggtctcagccctgtcgcccaggctggagtgcactagcacaacatcagctcactgcaacctccgcctcccaggttcaagcgattctcctgcctcagcctcccaagtagctgagactacaggcgcacgccagcatgtccagataattttttgtatttttagtagagatggggtttcaccatgttggccaggatggtctcaaatctcttgacctcgtgatctgcccatgtcggcttcccaaagtgttaggataacaggcatgagctaccgtgcccagcctacttaaaatattcttgaaatagctctccccacctccttttttttttttttttgagaatgagtttcactcgacacccaggctggagtgcagtggtgcgatcttggctcactgcaacctctgcctcccaggttcaagcgattatcctgcctcagcctcctgagtagctgggattacaaatgtgcaccaccacatctggctaattttttttttttttttttgtatttttagtagagacggggtttcaccaagttggcctggctggtctcgaacacctgacctcaattgatccacctgcctcggcctcccaaagtattataggcatgagccaccgagcccggccttttttgttttttgtttttttaaaggcagggttttgctctgttgcccaggctggagtgcagtggtgtgatcacagatcactgcagccttgacctctcctggtctcaagtgatcctcccacctcagccttcagaacagctgggactacaggtgtgtgtcaccatgcccagtaatttttttgtatatttgtagaggcagggtctcccaatgttgcctgggctggtctcaaactcctgggctcaagcaatccaccagctttggccttccaaagttctaggattatacgcatgagccactgtgccctgccccaatattttgttacttactagtgagactaaacacttttctaaaagtttgttagccatactatcctataaaagctgtttgttcatgtcttttgtccatttatctttttttttgtttttcttgagacagagtcttgctctgtggcccaggctggagtgcaggggtgcaatctcggctcactgcaagctccgcctcccaggttcaaatgattctcctgcctcagcctcctgagtagctgggattacaggcatgtgccaccatgcccagctaatttttttgtgtgtgtttttcagtagagatggggtttcaccatgttggccaggctgatctcgaattcctgacctcaggtgctccacccgcctcagcctcccaaagtactgggattacaggggtgagccaccgcacccggccaattttctgtatttttaatagagacagggtttcatcctgttggccaggctggcctcgaacttcggacctcaggtgatccacccgcctcgacctcccaaagtgctgggattacaggtgtgggccaccacacccagccaatttttttgtatttttagtagagacagggtttcatcatgttggccaggctggtcgcaaactcctgacctcaggtgatccacccgcctcagcatcccaaagtgctgggattacaggcatgagccaccactcccggccaatgttttgtatttttagtagagatggggtttcatcatgttggccagactggtctcaaactctggacctcaggtgatccacctgcctcagcctcccaaagtgtagggattacaggtgtgagccaccgcgcccagcctatgtttctattttatacatattcaacaaacatgattccccaacttctgcaaaataatttctttttcaagaacattgattttagagctcacactaagaaaaagaatacaaaaataatggcatagaaagtgaaaaaacaaaaataaaaagtagaaagctaaagtttcccattaaaatgatcaatatactgtgcagtaagtcaaatgtgtacaatgaattaagaaaatatgatatataaaaatccaaatttacaaaattaagtacaaataggtgtttatattacaaagtgatactggtttataaaaggattcaacatagattttttttaaatggttgttttcctcaatcaatttaacaatgattttaaatgtataaaattttaatatctctttgagacagtgatccaagcttcttcccttgatgatgttaccagttcatactttgtttcaataacctgtccctccacagaaagtaggtgcagtctcttcaccaatacactaagaagtactgtggtcaccatatatgcaaacctcaactctggacactcctgtgtgcctgagaatccaagtgaggaaaaagttttcattactaattcatcatcaaaccgatctggatcaaacttgtgtggagatggccaagtattaggatcctgaagtaccacaccaagggcataaaggacgagggtctgagctgctcaattttctctggagtaacaggaccatttccaaaaacttggtttatctcttcatataattttttttgaacttcttcagaggtggttaaaaaacagattgcccaggtacacaattttgcagttattatgcaactggccagagaaaatatcatactgtcttctaggatctgttggtcattaaggttcccttgtactaaggagtcaatgaaaatatgttgactgaagttccttccttttcgttcttttatgatgttccttaaaacagactccagttgcatgagggcatcttcatattgttttttccgagtcatgtttttatcaagtgacccatctagaaagccttttccaatctcagaccaaactgtgccatgattcttctggaagcgaatgacttcctgatcatcttcaaatgtactacccattaccatctgtgtaacagacttcatagcaaaaccaagcatatgctggctgaggggcacgtgctgggtctctgggtaggagagccatttatctaataattcttctgaaagctttaggaggagggcaaagttactcttcagagaatcagtcacaccattttcatacaattttttcctcatgtggttttcactcacactgccaccaccagattgataccttaataatgacttcagcatggtttcaaaagggtccgatgtcttattgggattgatatgctgcttcagtacatcaacagtgcccaaactaaccacgaggcgcctgccaaaccagaaggagaccacaggcccatatctctcatgcaaattaaccaggaactcatgcaaacttccactattcacaatatctggaagattaccatctttttcttcagttggagtaatccctggaattcctgcagcttgtctggaagccggatagaggtagagcacggctcccaccaacgccagcaagaaggtaacggcgaagatcgcgaagtccaacatggttctgccgcccagggagccacgtctcggatcggccgctccagc

SEQ ID NO: 15922 - RNA, 3795 nt, Homo sapiens
  source 1..3795: mol_type = other RNA
gctgggattacaggcatgagccatcacgcccggccaaagttttagaatttaagttattccaaaaaaaattttttttttcaaaaatacagactgcatccaattaaattctatgttaactggtaatgactaggtctaaaatgttaggtatttaccaataaatgacataaaataactcaacaacaaagggatttttttttttaagagatagggtctcactttatcactcaggtttggctgagggcagtggtgtgatcacagctcactgaagcctccaactcctgggctcaagtgatcctcccgcctcagtctaccagagtatattcttgaaagtaaaattacaaatgaaattcagcagtgttaaaaataagcccacttgcagacaattatcatttttcttcctttctttcctcactatctgtacttggcatatttcctacagtggctgtcttaaagaaaaaaaggaatccttcacaaatagtgtagccaaaaaagttggactaatatacaatgctatcagtaaagtattatatataaaatttataagtgctaaagtgtaattttgaaagacacttaagatactccttttttttttgagacaaggtctcagccctgtcgcccaggctggagtgcactagcacaacatcagctcactgcaacctccgcctcccaggttcaagcgattctcctgcctcagcctcccaagtagctgagactacaggcgcacgccagcatgtccagataattttttgtatttttagtagagatggggtttcaccatgttggccaggatggtctcaaatctcttgacctcgtgatctgcccatgtcggcttcccaaagtgttaggataacaggcatgagctaccgtgcccagcctacttaaaatattcttgaaatagctctccccacctccttttttttttttttttgagaatgagtttcactcgacacccaggctggagtgcagtggtgcgatcttggctcactgcaacctctgcctcccaggttcaagcgattatcctgcctcagcctcctgagtagctgggattacaaatgtgcaccaccacatctggctaattttttttttttttttttgtatttttagtagagacggggtttcaccaagttggcctggctggtctcgaacacctgacctcaattgatccacctgcctcggcctcccaaagtattataggcatgagccaccgagcccggccttttttgttttttgtttttttaaaggcagggttttgctctgttgcccaggctggagtgcagtggtgtgatcacagatcactgcagccttgacctctcctggtctcaagtgatcctcccacctcagccttcagaacagctgggactacaggtgtgtgtcaccatgcccagtaatttttttgtatatttgtagaggcagggtctcccaatgttgcctgggctggtctcaaactcctgggctcaagcaatccaccagctttggccttccaaagttctaggattatacgcatgagccactgtgccctgccccaatattttgttacttactagtgagactaaacacttttctaaaagtttgttagccatactatcctataaaagctgtttgttcatgtcttttgtccatttatctttttttttgtttttcttgagacagagtcttgctctgtggcccaggctggagtgcaggggtgcaatctcggctcactgcaagctccgcctcccaggttcaaatgattctcctgcctcagcctcctgagtagctgggattacaggcatgtgccaccatgcccagctaatttttttgtgtgtgtttttcagtagagatggggtttcaccatgttggccaggctgatctcgaattcctgacctcaggtgctccacccgcctcagcctcccaaagtactgggattacaggggtgagccaccgcacccggccaattttctgtatttttaatagagacagggtttcatcctgttggccaggctggcctcgaacttcggacctcaggtgatccacccgcctcgacctcccaaagtgctgggattacaggtgtgggccaccacacccagccaatttttttgtatttttagtagagacagggtttcatcatgttggccaggctggtcgcaaactcctgacctcaggtgatccacccgcctcagcatcccaaagtgctgggattacaggcatgagccaccactcccggccaatgttttgtatttttagtagagatggggtttcatcatgttggccagactggtctcaaactctggacctcaggtgatccacctgcctcagcctcccaaagtgtagggattacaggtgtgagccaccgcgcccagcctatgtttctattttatacatattcaacaaacatgattccccaacttctgcaaaataatttctttttcaagaacattgattttagagctcacactaagaaaaagaatacaaaaataatggcatagaaagtgaaaaaacaaaaataaaaagtagaaagctaaagtttcccattaaaatgatcaatatactgtgcagtaagtcaaatgtgtacaatgaattaagaaaatatgatatataaaaatccaaatttacaaaattaagtacaaataggtgtttatattacaaagtgatactggtttataaaaggattcaacatagattttttttaaatggttgttttcctcaatcaatttaacaatgattttaaatgtataaaattttaatatctctttgagacagtgatccaagcttcttcccttgatgatgttaccagttcatactttgtttcaataacctgtccctccacagaaagtaggtgcagtctcttcaccaatacactaagaagtactgtggtcaccatatatgcaaacctcaactctggacactcctgtgtgcctgagaatccaagtgaggaaaaagttttcattactaattcatcatcaaaccgatctggatcaaacttgtgtggagatggccaagtattaggatcctgaagtaccacaccaagggcataaaggacgagggtctgagctgctcaattttctctggagtaacaggaccatttccaaaaacttggtttatctcttcatataattttttttgaacttcttcagaggtggttaaaaaacagattgcccaggtacacaattttgcagttattatgcaactggccagagaaaatatcatactgtcttctaggatctgttggtcattaaggttcccttgtactaaggagtcaatgaaaatatgttgactgaagttccttccttttcgttcttttatgatgttccttaaaacagactccagttgcatgagggtgtgccatgattcttctggaagcgaatgacttcctgatcatcttcaaatgtactacccattaccatctgtgtaacagacttcatagcaaaaccaagcatatgctggctgaggggcacgtgctgggtctctgggtaggagagccatttatctaataattcttctgaaagctttaggaggagggcaaagttactcttcagagaatcagtcacaccattttcatacaattttttcctcatgtggttttcactcacactgccaccaccagattgataccttaataatgacttcagcatggtttcaaaagggtccgttttcttcagttggagtaatccctggaattcctgcagcttgtctggaagccggatagaggtagagcacggctcccaccaacgccagcaagaaggtaacggcgaagatcgcgaagtccaacatggttctgccgcccagggagccacgtctcggatcggccgctccagc

SEQ ID NO: 15923 - RNA, 1377 nt, Homo sapiens
  source 1..1377: mol_type = other RNA
gctgggattacaggcatgagccatcacgcctggctaattttgtatttttagtagagacagagtttctccacgttggtcaggctggtcctttttgttactcttatgggaattattcggcgggttaaaaaaatttttttttaataaatacatttttttttggccgggctcagtggctcacgcctgtaatcccagcactttgggaggccaaggcgggtggatcacctgaggtcaggagttcaaagccagcctgaccaacatggtgaaaccgagtctctactaaaaatacaaaaaattagccaggcgtggtagctcatgcctgtaatcccagctacttgggaggctgagacaggagaatcacttgaacccaagaagtggaggttgcagtgagccgagattgtgtcactgcactccagcctgggagacaagagcaaaactccgtcacaaaaccaaaccaaacctttttttcttttttttccaaaatgctactaagcaactacatctacccttggatgatagattaaaattggagtttaatatctgaattatttttacaaaagcagaaatagctaaataatgagtctcaggttaagtaggaggtggagtgggcgactatctaggaagaattcatcacctgatcagtgagtgacaatgcagaaggagctttgaaaactggctctatgagataacaactctgttgacatagaccttctctttctcctagaatcctttctcaaaggcatgcatgagtgcaccaaaaacgaattgccaggggaaagaaaagtaaaagctgactttctgtcatgagtagtgtgcaggccaggggctgcccgagaagcctctagcctctgcacactcagcagggatgcgtagtgtcctggctcgggtgtccccaagagaacgtgaggggcaggtcccagagcagggcccaggagacagagactgattcatttggatgaggagcacttgccaccccttgaggagacaccttgagggagcggaccctccccccagtggtcaccccctcctgaggatcgctgcccttggttgatgccctggtctctgccctttccccctgggccattttcctgccgacctcccacctcctggggcagaagatggaggggtgggggtccttcctctggctcttcagcttcggaagcagactcagtagactcatcgtcgtagaagtcaatcgtggcttgcactgggaaactggccagtacttgctccccggaactccgcaggtattcttgacgctttgacatgggtaaatagactcggccttccagttctggtcagctcagcatctccaggtgtctggatccaaggtcgccacggcgcggggctgctgggcttcccctgccggatgtgggatgt

SEQ ID NO: 15924 - RNA, 1588 nt, Homo sapiens
  source 1..1588: mol_type = other RNA
gctgggattacaggcatgagccatcacgcctggctaattttgtatttttagtagagacagagtttctccacgttggtcaggctggtcctttttgttactcttatgggaattattcggcgggttaaaaaaatttttttttaataaatacatttttttttggccgggctcagtggctcacgcctgtaatcccagcactttgggaggccaaggcgggtggatcacctgaggtcaggagttcaaagccagcctgaccaacatggtgaaaccgagtctctactaaaaatacaaaaaattagccaggcgtggtagctcatgcctgtaatcccagctacttgggaggctgagacaggagaatcacttgaacccaagaagtggaggttgcagtgagccgagattgtgtcactgcactccagcctgggagacaagagcaaaactccgtcacaaaaccaaaccaaacctttttttcttttttttccaaaatgctactaagcaactacatctacccttggatgatagattaaaattggagtttaatatctgaattatttttacaaaagcagaaatagctaaataatgagtctcaggttaagtaggaggtggagtgggcgactatctaggaagaattcatcacctgatcagtgagtgacaatgcagaaggagctttgaaaactggctctatgagataacaactctgttgacatagaccttctctttctcctagaatcctttctcaaaggcatgcatgagtgcaccaaaaacgaattgccaggggaaagaaaagtaaaagctgactttctgtcatgagtagtgtgcaggccaggggctgcccgagaagcctctagcctctgcacactcagcagggatgcgtagtgtcctggctcgggtgtccccaagagaacgtgaggggcaggtcccagagcagggcccaggagacagagactgattcatttggatgaggagcacttgccaccccttgaggagacaccttgagggagcggaccctccccccagtggtcaccccctcctgaggatcgctgcccttggttgatgccctggtctctgccctttccccctgggccattttcctgccgacctcccacctcctggggcagaagatggaggggtgggggtccttcctctggctcttcagcttcggaagcagactcagtagactcatcgtcgtagaagtcaatcgtggcttgcactgggaaactggccagtacttgctccccggaactccgcaggtattcttgacgctttgacatgggtaaatagactcttacaggatgctgaaacccaaaggctccctttgatccaaaagtgtgttggtcagccctaggttcaagcggccttccagttctggtcagctcagcatctccaggtgtctggatccaaggtcgccacggcgcggggctctccggcccgcgcggtggcggaggcctccagggagcgtccccggggcagtgacagccgcgcccccgcgccttccgggctccggccgccgcttcgggctccatggtgccggcggagcccgcgccccttgctgcggcgccggcctacgagcgcgcctagatccactcgggctaac

SEQ ID NO: 15925 - RNA, 1497 nt, Homo sapiens
  source 1..1497: mol_type = other RNA
gctgggattacaggcatgagccatcacgcctggctaattttgtatttttagtagagacagagtttctccacgttggtcaggctggtcctttttgttactcttatgggaattattcggcgggttaaaaaaatttttttttaataaatacatttttttttggccgggctcagtggctcacgcctgtaatcccagcactttgggaggccaaggcgggtggatcacctgaggtcaggagttcaaagccagcctgaccaacatggtgaaaccgagtctctactaaaaatacaaaaaattagccaggcgtggtagctcatgcctgtaatcccagctacttgggaggctgagacaggagaatcacttgaacccaagaagtggaggttgcagtgagccgagattgtgtcactgcactccagcctgggagacaagagcaaaactccgtcacaaaaccaaaccaaacctttttttcttttttttccaaaatgctactaagcaactacatctacccttggatgatagattaaaattggagtttaatatctgaattatttttacaaaagcagaaatagctaaataatgagtctcaggttaagtaggaggtggagtgggcgactatctaggaagaattcatcacctgatcagtgagtgacaatgcagaaggagctttgaaaactggctctatgagataacaactctgttgacatagaccttctctttctcctagaatcctttctcaaaggcatgcatgagtgcaccaaaaacgaattgccaggggaaagaaaagtaaaagctgactttctgtcatgagtagtgtgcaggccaggggctgcccgagaagcctctagcctctgcacactcagcagggatgcgtagtgtcctggctcgggtgtccccaagagaacgtgaggggcaggtcccagagcagggcccaggagacagagactgattcatttggatgaggagcacttgccaccccttgaggagacaccttgagggagcggaccctccccccagtggtcaccccctcctgaggatcgctgcccttggttgatgccctggtctctgccctttccccctgggccattttcctgccgacctcccacctcctggggcagaagatggaggggtgggggtccttcctctggctcttcagcttcggaagcagactcagtagactcatcgtcgtagaagtcaatcgtggcttgcactgggaaactggccagtacttgctccccggaactccgcaggtattcttgacgctttgacatgggtaaatagactcttacaggatgctgaaacccaaaggctccctttgatccaaaagtgtgttggtcagccctaggttcaagcggccttccagttctggtcagctcagcatctccaggtgtctggatccaaggtcgccacggcgcggggctgctgggcttcccctgccggatgtgggatgtgaggagtcccggcttctccgtccctctgtggtccccgcggcctcgggctttg

SEQ ID NO: 15926 - RNA, 503 nt, Homo sapiens
  source 1..503: mol_type = other RNA
gctgggattacaggcatgagccatcacgcttggcctccccttgaatttaaaccaaaaaaaacaaaaacagacacaagtgtaagttggttacaaaatcttttccaaaatatcttctcttactaaagtttccttcatgtaaatagtgtttggaatagaaagagggtggtgacaaaataatcttcctgtatcttatatcaagtttaaatagacagtggaagccaatttgggattcataaatgcagtactatgacacttagagaaataaaaaacttttagaaagcatctttaggaaattctaaggttaaattccgttgaactggggaacaaataaagctaaggtaaagtctggtattttctcattcagtaataaagaaccacaacgtgcagattcttcacctgccaagcaaacagttctaaaaacccctcttggtaggaaaggagataaaaaattatatttaagaacacctggttgggcacagtggctcacgcctgtaatcccagca

SEQ ID NO: 15927 - RNA, 2427 nt, Homo sapiens
  source 1..2427: mol_type = other RNA
gctgggattacaggcatgagccatcatacctggccatctccttcttctaacttatcttctcctttagccttgacctcgaggtatggtccatggaccagcagcatcggcaccatctgggaacttgttagaaatgcagaagttcccccatcaccgcccactccctgccccagtcagaacctgcattttaccaagaccccagctgattcctgtgcataggaaagatggaaaagggctgctctgtagtagtgtggaccactgcctgacaccgcatcattatctgtttgttgtctacctttggtgagggcagggatcatgtctgtcttgttctctgttgtatgcccagggacaaaaagtgtaagtgtctgacacataccaggagctcaataaacacttgttaaatgattgacagactgaatgaatgaatgagccagaaatcaaacccaagcctcctaattaaactgattcacaattctgtgcttgtttgttcagtgactcatttccaggtagagctgggattcagtaactccagatctcctctccattctgaatgatggaatcacacttggttcctacctcacagggggtttgtgaggacagttcctattccaagtgctttcccacttgatttccccaaaactccatgacacaggaaggcacatactaggttattcccatttttcagatgtgaaaattgaggcccagagaagttgaggctcttgcctgagatcatacaactcagaagtggtagaaccaggatttgaactcatacctcctgattgcaaatcaagttctcatccctagtccatgttcattcatttgttcattcattccacagtcaagtaccagccccaggctgggagctgggagggcatgaataaagttaactaagaagtcttggaacccaaagggctccccaggccagatggatatataaggaatggtgattccgtgtgcccagtgcttctgtggactcaaaaacctgcagaagcatgaaggtgggctcaactaatctgcttggaggcatctcagaagacttcccagaggaggtgatgtgtgaaatttcatcagggtggggcagcaggaggagcatcccaagtggagagaccagagcatgaaaaggcctggaagtgtgaaggtgcctaagcacatccccaaggtctatgtgctcagaggaaggtgatccaggtccatgagccggggtgaggggtggtgaaggatgaggctggggagggaggccaggcctgcctgccagaggcctggaatggcaagatggtggtggcccttacccacgtgccagctgtactcctaggatgacatgactgggtactggaacttctcctcgggcttcagccgatgccgtgcctggaggtccagggcgtggccttggccatcgtgggagatgcctgggaagagcagctgcaggattcttggggagacctgcctcatttctaaactctccggcctggtctgacctgctggcccctgagttgcttttctggccttccagactctgtctcccttgggtggggagtcctggacacccactcccttggacagctggttctgggcccccttggtctctggccatccaacctgtacctccttgctatcacgggagctggtggcaggcactgggcccgctaccaaggctgacctggatggggcctgctggagctgcttcctgggcacggtcccctcccttaggtacttgtggccatcgttgatcttccaggcaacttgggtggtggcctccttttggatgcattccttccagcaggcctggttctgggaggtccacagctccccaggggcagggagaggtggaggagggaagaatggctcttcccacagctctgcggcctgtgtttgggctcccagagcctcatctccaaggatacatgcagccgatgagggctgggttgccaaggccctgaaagagaggagaggctgggctgccctgggggacttggggggtcccacaggcagaagaacagaccaggctggaaaagggtgcagagcctggccacaacccacccaaggtgcctgtccttcccccgagggacgggcccaggcctttaccttcacacccacagggctctggggtggcgcacggggtgctgcagcctctattccattcagcaaactctgatgcacacctactatgtgccaggcacccaatgggggtccaaaaagaggcccagtcttccccggcctcagggagcgctggacacgcagctgaggaggtttccagggcaactctagggtccagctcctcagatacgcagctctgtcccttgctagcggagtggcctcatcagcgcagaagaagagaggtgggtgggtccccctcctcctggtctgggagagcccgcgccttccccaccgcagggactccgctttctggccactccctgaggccaccaacat

SEQ ID NO: 15928 - RNA, 3519 nt, Homo sapiens
  source 1..3519: mol_type = other RNA
gctgggattacaggcatgagccatcatgccctgcctgtagttcacttttaagtatattttttaaaagtaaaaaatctgaagcagctgccacccaagtgtagaatagataaattgtgatataatcatagaatgaaaccagacataaccatgaagagaactgaactactgctagacaggacaacgtggatgaatctcacatgcaggatgctgatccggacaccacaagaaaaaacaaaagaaggtgcctactgagttttcttctttccagatgaccaactcttaacttactcatctgtttttttcactgttctgcttcttttgaagaagatttgaggtgacttacaaaggtgtatggcatatttataactgaagaaatctgggtgatgttaaaacgagggcaggaaaataaggtggaaaccagatgtaaggatagtcttcactatttatgtcaggaattcctacaaactttctatggtgaacagaatagagcttcctagcagtcaatgcaaagaagaaacacaacaattccacaccccaaagttaacagtcttgcttatcagaagcacaggtagttctgaaatctgatagaaaatgttcctgtatcatttcagaacacgcaactatgtgatcaaacccctttctatttgtttaaaaatttgtcaaacatcccatgtttgaccctggatgtctgaatcccctcagcccacattttcccccctacaccatgcccacaccatccccatagaatttagggtgaggcagcatctcagtgattgacaggcccctccttagaccccgtttactttcctgggtgtggtttggggtaagccctgttcatgaaggctggatttctgttctttgggttgcccagcttgccaccctcatttctggaacccagaccagcatcctcagcccacgctttgccactcagctcatcttcttcccagttggcacttctcagtgaccccatcccttccccagcagtgactctgcgtggggcagctccctggtggctggactctttccattttggcatttgggttagtggatctttccactttctggctccagtttttgagttgaattcatatgtttccccggtcactggatctatggcttctccatcaaagatagtgttcatctggatagtttccaccacgacgtctctctctgcagtcttcgtttagaggttccttgttcttcccagtcttgcaggggcagtgtctgtggatggctttggccaataggacgaccaggtacacgaggagacccagaagcaatatggagcccaaagtgatgacaaacggcacgtaccatgcagatggagagtaaacgtttttcctcaggacctgataggtgaccctgggcctgggggtcgtggtgatgatagtggttgggtggggaatgactttaatactcagtgtcactgttcctgtctcaacaagagcctccgctttcttcctgtcagacatcaagttgtcatcagttacgtagacaagtagcttgtagtcccagatcttatcaaacccaccagcatagtcaaagcgagatgtaagcagcaggcgtgtgacattggaaccagcattgggagagaaggtgaaatgattgttgacgttacctgggccaatggaataacggaaagatctggggctggaatcaaggtcggtacatgtcagcttgaaattctgaatatttgtgccaactttcagatccactgggagggccaggaaataagagtttggagtacaaattggcttttcatcattttcttcaaggatgttcacagtaacagtgacagagcttgtgtcttcgttgttggtggcctggattctgagaatatagatgggggttgtttcacagtccactttagttaccagctggagttctcctgtcttgggattaatccaaaatacatttggatactggaggctggcccctccagtggagatggagtacaggaggctgctctgggggaggtctttatcagtggctcgcacctgtcccactcgggttctggcgggccttctttctgacacatcaaatacataggatggcctatcaaaaatgagaggaaactcattttctgggcttgttaggatataaacgtagacgttatttttatagtaagggggggccacatcctgcacctggattatcaccgtatatttattgccggctgctaggttacttggattttcgtagtctagatcaccaatcagcacaatcttcccagagccagctggatcctgtaaaaatctgctgccgctccccactccagatggcatggtgaagttgaatctgttgtttggtgcctcactgtcatcatcaaagcagaacttgtttaggtcaagaagcaacgtccccttggctgttctttccggcaccataatgctgaaggtgaacttttggcatgtggcaggattgtcgttgacgtcttccacaatgaaggttatctggatgcgattctcctgacccccatatggtctgtccttcactagaacttccagggaaatggtgggattttgtctcaattcacctgcatctcggtctatcctttgggccacttggattgtaccagtcaactgatttatcatgaaatatttgctaacagtggtaatgctgtagaggaggtggctgggaaaaccttcatcatcaggatcctccgctgtgatattggccacgatggttcctggactcagttcctccaggactgtgtacactcgtgtcgggctggtaaagcgagggacttcgtcgttgaggttcacgatgttcacctggagctctgtggaggctttgaggcctccactgtccctcacctccacgatgagatggaaacttctgtgtcctgcttcaaagtccaattctgttgtggagaagagggtgccattagcagacattctgaagctctttgggggagaaatcaggaaataactgaggggaatgtttcggcttgtgtcttctggatcgaaggcctcaacctggtaaatgaatccagggtttgctctttctactatgtagaggtgtagaccttctgccaagttgccttgaaactgaggtggctcgttcacatctgttacctggacagtcaggacttgcaggtctgtgacaccaacctcatccttcacataaatctgcaaatcaaatatgtttggtcctgtttcaaaatctagttgttccatcccagtggtgacaacctcaaagtaggtgcctgacagccaattcaccctaaaagcttcagtgaggggatttgagttgactatctggggaaatcctgggatcacaggtgacaatgatgctgataacttcacagaaaacttgtgcactgaagtcccaggtggagaattctctgccacattgcctgtagcaggtaagaggattaggtgtagtgcttctccccctgacatggcacccaggagagccaggagaatgattgcttcctgcatacttgatggtcacaactgtgcgtgcttccagcacattagccacagcctgaatcccgtctcacacccaaagtttatt

SEQ ID NO: 15929 - RNA, 3268 nt, Homo sapiens
  source 1..3268: mol_type = other RNA
gctgggattacaggcatgagccatcatgccctgcctgtagttcacttttaagtatattttttaaaagtaaaaaatctgaagcagctgccacccaagtgtagaatagataaattgtgatataatcatagaatgaaaccagacataaccatgaagagaactgaactactgctagacaggacaacgtggatgaatctcacatgcaggatgctgatccggacaccacaagaaaaaacaaaagaaggtgcctactgagttttcttctttccagatgaccaactcttaacttactcatctgtttttttcactgttctgcttcttttgaagaagatttgaggtgacttacaaaggtgtatggcatatttataactgaagaaatctgggtgatgttaaaacgagggcaggaaaataaggtggaaaccagatgtaaggatagtcttcactatttatgtcaggaattcctacaaactttctatggtgaacagaatagagcttcctagcagtcaatgcaaagaagaaacacaacaattccacaccccaaagttaacagtcttgcttatcagaagcacaggtagttctgaaatctgatagaaaatgttcctgtatcatttcagaacacgcaactatgtgatcaaacccctttctatttgtttaaaaatttgtcaaacatcccatgtttgaccctggatgtctgaatcccctcagcccacattttcccccctacaccatgcccacaccatccccatagaatttagggtgaggcagcatctcagtgattgacaggcccctccttagaccccgtttactttcctgggtgtggtttggggtaagccctgttcatgaaggctggatttctgttctttgggttgcccagcttgccaccctcatttctggaacccagaccagcatcctcagcccacgctttgccactcagctcatcttcttcccagttggcacttctcagtgaccccatcccttccccagcagtgactctgcgtggggcagctccctggtggctggactctttccattttggcatttgggttagtggatctttccactttctggctccagtttttgagttgaattcatatgtttccccggtcactggatctatggcttctccatcaaagatagtgttcatctggatagtttccaccacgacgtctctctctgcagtcttcgtttagaggttccttgttcttcccagtcttgcaggggcagtgtctgtggatggctttggccaataggacgaccaggtacacgaggagacccagaagcaatatggagcccaaagtgatgacaaacggcacgtaccatgcagatggagagtaaacgtttttcctcaggacctgataggtgaccctgggctgggccaatggaataacggaaagatctggggctggaatcaaggtcggtacatgtcagcttgaaattctgaatatttgtgccaactttcagatccactgggagggccaggaaataagagtttggagtacaaattggcttttcatcattttcttcaaggatgttcacagtaacagtgacagagcttgtgtcttcgttgttggtggcctggattctgagaatatagatgggggttgtttcacagtccactttagttaccagctggagttctcctgtcttgggattaatccaaaatacatttggatactggaggctggcccctccagtggagatggagtacaggaggctgctctgggggaggtctttatcagtggctcgcacctgtcccactcgggttctggcgggccttctttctgacacatcaaatacataggatggcctatcaaaaatgagaggaaactcattttctgggcttgttaggatataaacgtagacgttatttttatagtaagggggggccacatcctgcacctggattatcaccgtatatttattgccggctgctaggttacttggattttcgtagtctagatcaccaatcagcacaatcttcccagagccagctggatcctgtaaaaatctgctgccgctccccactccagatggcatggtgaagttgaatctgttgtttggtgcctcactgtcatcatcaaagcagaacttgtttaggtcaagaagcaacgtccccttggctgttctttccggcaccataatgctgaaggtgaacttttggcatgtggcaggattgtcgttgacgtcttccacaatgaaggttatctggatgcgattctcctgacccccatatggtctgtccttcactagaacttccagggaaatggtgggattttgtctcaattcacctgcatctcggtctatcctttgggccacttggattgtaccagtcaactgatttatcatgaaatatttgctaacagtggtaatgctgtagaggaggtggctgggaaaaccttcatcatcaggatcctccgctgtgatattggccacgatggttcctggactcagttcctccaggactgtgtacactcgtgtcgggctggtaaagcgagggacttcgtcgttgaggttcacgatgttcacctggagctctgtggaggctttgaggcctccactgtccctcacctccacgatgagatggaaacttctgtgtcctgcttcaaagtccaattctgttgtggagaagagggtgccattagcagacattctgaagctctttgggggagaaatcaggaaataactgaggggaatgtttcggcttgtgtcttctggatcgaaggcctcaacctggtaaatgaatccagggtttgctctttctactatgtagaggtgtagaccttctgccaagttgccttgaaactgaggtggctcgttcacatctgttacctggacagtcaggacttgcaggtctgtgacaccaacctcatccttcacataaatctgcaaatcaaatatgtttggtcctgtttcaaaatctagttgttccatcccagtggtgacaacctcaaagtaggtgcctgacagccaattcaccctaaaagcttcagtgaggggatttgagttgactatctggggaaatcctgggatcacaggtgacaatgatgctgataacttcacagaaaacttgtgcactgaagtcccaggtggagaattctctgccacattgcctgtagcaggtaagaggattaggtgtagtgcttctccccctgacatggcacccaggagagccaggagaatgattgcttcctgcatacttgatggtcacaactgtgcgtgcttccagcacattagccacagcctgaatcccgtctcacacccaaagtttatt

SEQ ID NO: 15930 - RNA, 3681 nt, Homo sapiens
  source 1..3681: mol_type = other RNA
gctgggattacaggcatgagccatcatgccctgcctgtagttcacttttaagtatattttttaaaagtaaaaaatctgaagcagctgccacccaagtgtagaatagataaattgtgatataatcatagaatgaaaccagacataaccatgaagagaactgaactactgctagacaggacaacgtggatgaatctcacatgcaggatgctgatccggacaccacaagaaaaaacaaaagaaggtgcctactgagttttcttctttccagatgaccaactcttaacttactcatctgtttttttcactgttctgcttcttttgaagaagatttgaggtgacttacaaaggtgtatggcatatttataactgaagaaatctgggtgatgttaaaacgagggcaggaaaataaggtggaaaccagatgtaaggatagtcttcactatttatgtcaggaattcctacaaactttctatggtgaacagaatagagcttcctagcagtcaatgcaaagaagaaacacaacaattccacaccccaaagttaacagtcttgcttatcagaagcacaggtagttctgaaatctgatagaaaatgttcctgtatcatttcagaacacgcaactatgtgatcaaacccctttctatttgtttaaaaatttgtcaaacatcccatgtttgaccctggatgtctgaatcccctcagcccacattttcccccctacaccatgcccacaccatccccatagaatttagggtgaggcagcatctcagtgattgacaggcccctccttagaccccgtttactttcctgggtgtggtttggggtaagccctgttcatgaaggctggatttctgttctttgggttgcccagcttgccaccctcatttctggaacccagaccagcatcctcagcccacgctttgccactcagctcatcttcttcccagttggcacttctcagtgaccccatcccttccccagcagtgactctgcgtggggcagctccctggtggctggactctttccattttggcatttgggttagtggatctttccactttctggctccagtttttgagttgaattcatatgtttccccggtcactggatctatggcttctccatcaaagatagtgttcatctggatagtttccaccacgacgtctctctctgcagtcttcgtttctccgcttccttccagccacagaagatgcagctgaaaatgctccaagatgtgatcgcggcctgattctttgccgagtaggaacctttttacgtagcacaacagagcaagcaaaaaacaacagacaagggaaacaggtactgtacatacctcctttctttgtcagaggttccttgttcttcccagtcttgcaggggcagtgtctgtggatggctttggccaataggacgaccaggtacacgaggagacccagaagcaatatggagcccaaagtgatgacaaacggcacgtaccatgcagatggagagtaaacgtttttcctcaggacctgataggtgaccctgggcctgggggtcgtggtgatgatagtggttgggtggggaatgactttaatactcagtgtcactgttcctgtctcaacaagagcctccgctttcttcctgtcagacatcaagttgtcatcagttacgtagacaagtagcttgtagtcccagatcttatcaaacccaccagcatagtcaaagcgagatgtaagcagcaggcgtgtgacattggaaccagcattgggagagaaggtgaaatgattgttgacgttacctgggccaatggaataacggaaagatctggggctggaatcaaggtcggtacatgtcagcttgaaattctgaatatttgtgccaactttcagatccactgggagggccaggaaataagagtttggagtacaaattggcttttcatcattttcttcaaggatgttcacagtaacagtgacagagcttgtgtcttcgttgttggtggcctggattctgagaatatagatgggggttgtttcacagtccactttagttaccagctggagttctcctgtcttgggattaatccaaaatacatttggatactggaggctggcccctccagtggagatggagtacaggaggctgctctgggggaggtctttatcagtggctcgcacctgtcccactcgggttctggcgggccttctttctgacacatcaaatacataggatggcctatcaaaaatgagaggaaactcattttctgggcttgttaggatataaacgtagacgttatttttatagtaagggggggccacatcctgcacctggattatcaccgtatatttattgccggctgctaggttacttggattttcgtagtctagatcaccaatcagcacaatcttcccagagccagctggatcctgtaaaaatctgctgccgctccccactccagatggcatggtgaagttgaatctgttgtttggtgcctcactgtcatcatcaaagcagaacttgtttaggtcaagaagcaacgtccccttggctgttctttccggcaccataatgctgaaggtgaacttttggcatgtggcaggattgtcgttgacgtcttccacaatgaaggttatctggatgcgattctcctgacccccatatggtctgtccttcactagaacttccagggaaatggtgggattttgtctcaattcacctgcatctcggtctatcctttgggccacttggattgtaccagtcaactgatttatcatgaaatatttgctaacagtggtaatgctgtagaggaggtggctgggaaaaccttcatcatcaggatcctccgctgtgatattggccacgatggttcctggactcagttcctccaggactgtgtacactcgtgtcgggctggtaaagcgagggacttcgtcgttgaggttcacgatgttcacctggagctctgtggaggctttgaggcctccactgtccctcacctccacgatgagatggaaacttctgtgtcctgcttcaaagtccaattctgttgtggagaagagggtgccattagcagacattctgaagctctttgggggagaaatcaggaaataactgaggggaatgtttcggcttgtgtcttctggatcgaaggcctcaacctggtaaatgaatccagggtttgctctttctactatgtagaggtgtagaccttctgccaagttgccttgaaactgaggtggctcgttcacatctgttacctggacagtcaggacttgcaggtctgtgacaccaacctcatccttcacataaatctgcaaatcaaatatgtttggtcctgtttcaaaatctagttgttccatcccagtggtgacaacctcaaagtaggtgcctgacagccaattcaccctaaaagcttcagtgaggggatttgagttgactatctggggaaatcctgggatcacaggtgacaatgatgctgataacttcacagaaaacttgtgcactgaagtcccaggtggagaattctctgccacattgcctgtagcaggtaagaggattaggtgtagtgcttctccccctgacatggcacccaggagagccaggagaatgattgcttcctgcatacttgatggtcacaactgtgcgtgcttccagcacattagccacagcctgaatcccgtctcacacccaaagtttatt

SEQ ID NO: 15931 - RNA, 3149 nt, Homo sapiens
  source 1..3149: mol_type = other RNA
gctgggattacaggcatgagccatcatgccctgcctgtagttcacttttaagtatattttttaaaagtaaaaaatctgaagcagctgccacccaagtgtagaatagataaattgtgatataatcatagaatgaaaccagacataaccatgaagagaactgaactactgctagacaggacaacgtggatgaatctcacatgcaggatgctgatccggacaccacaagaaaaaacaaaagaaggtgcctactgagttttcttctttccagatgaccaactcttaacttactcatctgtttttttcactgttctgcttcttttgaagaagatttgaggtgacttacaaaggtgtatggcatatttataactgaagaaatctgggtgatgttaaaacgagggcaggaaaataaggtggaaaccagatgtaaggatagtcttcactatttatgtcaggaattcctacaaactttctatggtgaacagaatagagcttcctagcagtcaatgcaaagaagaaacacaacaattccacaccccaaagttaacagtcttgcttatcagaagcacaggtagttctgaaatctgatagaaaatgttcctgtatcatttcagaacacgcaactatgtgatcaaacccctttctatttgtttaaaaatttgtcaaacatcccatgtttgaccctggatgtctgaatcccctcagcccacattttcccccctacaccatgcccacaccatccccatagaatttagggtgaggcagcatctcagtgattgacaggcccctccttagaccccgtttactttcctgggtgtggtttggggtaagccctgttcatgaaggctggatttctgttctttgggttgcccagcttgccaccctcatttctggaacccagaccagcatcctcagcccacgctttgccactcagctcatcttcttcccagttggcacttctcagtgaccccatcccttccccagcagtgactctgcgtggggcagctccctggtggctggactctttccattttggcatttgggttagtggatctttccactttctggctccagtttttgagttgaattcatatgtttccccggtcactggatctatggcttctccatcaaagatagtgttcatctggatagtttccaccacgacgtctctctctgcagtcttcgtttctcctttctttgtcagaggttccttgttcttcccagtcttgcaggggcagtgtctgtggatggctttggccaataggacgaccaggtacacgaggagacccagaagcaatatggagcccaaagtgatgacaaacggcacgtaccatgcagatggagagtaaacgtttttcctcaggacctgataggtgaccctgggcctgggggtcgtggtgatgatagtggttgggtggggaatgactttaatactcagtgtcactgttcctgtctcaacaagagcctccgctttcttcctgggccaatggaataacggaaagatctggggctggaatcaaggtcggtacatgtcagcttgaaattctgaatatttgtgccaactttcagatccactgggagggccaggaaataagagtttggagtacaaattggcttttcatcattttcttcaaggatgttcacagtaaccgggccttctttctgacacatcaaatacataggatggcctatcaaaaatgagaggaaactcattttctgggcttgttaggatataaacgtagacgttatttttatagtaagggggggccacatcctgcacctggattatcaccgtatatttattgccggctgctaggttacttggattttcgtagtctagatcaccaatcagcacaatcttcccagagccagctggatcctgtaaaaatctgctgccgctccccactccagatggcatggtgaagttgaatctgttgtttggtgcctcactgtcatcatcaaagcagaacttgtttaggtcaagaagcaacgtccccttggctgttctttccggcaccataatgctgaaggtgaacttttggcatgtggcaggattgtcgttgacgtcttccacaatgaaggttatctggatgcgattctcctgacccccatatggtctgtccttcactagaacttccagggaaatggtgggattttgtctcaattcacctgcatctcggtctatcctttgggccacttggattgtaccagtcaactgatttatcatgaaatatttgctaacagtggtaatgctgtagaggaggtggctgggaaaaccttcatcatcaggatcctccgctgtgatattggccacgatggttcctggactcagttcctccaggactgtgtacactcgtgtcgggctggtaaagcgagggacttcgtcgttgaggttcacgatgttcacctggagctctgtggaggctttgaggcctccactgtccctcacctccacgatgagatggaaacttctgtgtcctgcttcaaagtccaattctgttgtggagaagagggtgccattagcagacattctgaagctctttgggggagaaatcaggaaataactgaggggaatgtttcggcttgtgtcttctggatcgaaggcctcaacctggtaaatgaatccagggtttgctctttctactatgtagaggtgtagaccttctgccaagttgccttgaaactgaggtggctcgttcacatctgttacctggacagtcaggacttgcaggtctgtgacaccaacctcatccttcacataaatctgcaaatcaaatatgtttggtcctgtttcaaaatctagttgttccatcccagtggtgacaacctcaaagtaggtgcctgacagccaattcaccctaaaagcttcagtgaggggatttgagttgactatctggggaaatcctgggatcacaggtgacaatgatgctgataacttcacagaaaacttgtgcactgaagtcccaggtggagaattctctgccacattgcctgtagcaggtaagaggattaggtgtagtgcttctccccctgacatggcacccaggagagccaggagaatgattgcttcctgcatacttgatggtcacaactgtgcgtgcttccagcacattagccacagcctgaatcccgtctcacacccaaagtttatt

SEQ ID NO: 15932 - RNA, 3134 nt, Homo sapiens
  source 1..3134: mol_type = other RNA
gctgggattacaggcatgagccatcatgccctgcctgtagttcacttttaagtatattttttaaaagtaaaaaatctgaagcagctgccacccaagtgtagaatagataaattgtgatataatcatagaatgaaaccagacataaccatgaagagaactgaactactgctagacaggacaacgtggatgaatctcacatgcaggatgctgatccggacaccacaagaaaaaacaaaagaaggtgcctactgagttttcttctttccagatgaccaactcttaacttactcatctgtttttttcactgttctgcttcttttgaagaagatttgaggtgacttacaaaggtgtatggcatatttataactgaagaaatctgggtgatgttaaaacgagggcaggaaaataaggtggaaaccagatgtaaggatagtcttcactatttatgtcaggaattcctacaaactttctatggtgaacagaatagagcttcctagcagtcaatgcaaagaagaaacacaacaattccacaccccaaagttaacagtcttgcttatcagaagcacaggtagttctgaaatctgatagaaaatgttcctgtatcatttcagaacacgcaactatgtgatcaaacccctttctatttgtttaaaaatttgtcaaacatcccatgtttgaccctggatgtctgaatcccctcagcccacattttcccccctacaccatgcccacaccatccccatagaatttagggtgaggcagcatctcagtgattgacaggcccctccttagaccccgtttactttcctgggtgtggtttggggtaagccctgttcatgaaggctggatttctgttctttgggttgcccagcttgccaccctcatttctggaacccagaccagcatcctcagcccacgctttgccactcagctcatcttcttcccagttggcacttctcagtgaccccatcccttccccagcagtgactctgcgtggggcagctccctggtggctggactctttccattttggcatttgggttagtggatctttccactttctggctccagtttttgagttgaattcatatgtttccccggtcactggatctatggcttctccatcaaagatagtgttcatctggatagtttccaccacgacgtctctctctgcagtcttcgtttctcctttctttgtcagaggttccttgttcttcccagtcttgcaggggcagtgtctgtggatggctttggccaataggacgaccaggtacacgaggagacccagaagcaatatggagcccaaagtgatgacaaacggcacgtaccatgcagatggagagtaaacgtttttcctcaggacctgataggtgaccctgggcctgggggtcgtggtgatgatagtggttgggtggggaatgactttaatactcagtgtcactgttcctgtctcaacaagagcctccgctttcttcctgtcagacatcaagttgtcatcagttacgtagacaagtagcttgtagtcccagatcttatcaaacccaccagcatagtcaaagcgagatgtaagcagcaggcgtgtgacattggaaccagcattgggagagaaggtgaaatgattgttgacgttaccgggccttctttctgacacatcaaatacataggatggcctatcaaaaatgagaggaaactcattttctgggcttgttaggatataaacgtagacgttatttttatagtaagggggggccacatcctgcacctggattatcaccgtatatttattgccggctgctaggttacttggattttcgtagtctagatcaccaatcagcacaatcttcccagagccagctggatcctgtaaaaatctgctgccgctccccactccagatggcatggtgaagttgaatctgttgtttggtgcctcactgtcatcatcaaagcagaacttgtttaggtcaagaagcaacgtccccttggctgttctttccggcaccataatgctgaaggtgaacttttggcatgtggcaggattgtcgttgacgtcttccacaatgaaggttatctggatgcgattctcctgacccccatatggtctgtccttcactagaacttccagggaaatggtgggattttgtctcaattcacctgcatctcggtctatcctttgggccacttggattgtaccagtcaactgatttatcatgaaatatttgctaacagtggtaatgctgtagaggaggtggctgggaaaaccttcatcatcaggatcctccgctgtgatattggccacgatggttcctggactcagttcctccaggactgtgtacactcgtgtcgggctggtaaagcgagggacttcgtcgttgaggttcacgatgttcacctggagctctgtggaggctttgaggcctccactgtccctcacctccacgatgagatggaaacttctgtgtcctgcttcaaagtccaattctgttgtggagaagagggtgccattagcagacattctgaagctctttgggggagaaatcaggaaataactgaggggaatgtttcggcttgtgtcttctggatcgaaggcctcaacctggtaaatgaatccagggtttgctctttctactatgtagaggtgtagaccttctgccaagttgccttgaaactgaggtggctcgttcacatctgttacctggacagtcaggacttgcaggtctgtgacaccaacctcatccttcacataaatctgcaaatcaaatatgtttggtcctgtttcaaaatctagttgttccatcccagtggtgacaacctcaaagtaggtgcctgacagccaattcaccctaaaagcttcagtgaggggatttgagttgactatctggggaaatcctgggatcacaggtgacaatgatgctgataacttcacagaaaacttgtgcactgaagtcccaggtggagaattctctgccacattgcctgtagcaggtaagaggattaggtgtagtgcttctccccctgacatggcacccaggagagccaggagaatgattgcttcctgcatacttgatggtcacaactgtgcgtgcttccagcacattagccacagcctgaatcccgtctcacacccaaagtttatt

SEQ ID NO: 15933 - RNA, 3317 nt, Homo sapiens
  source 1..3317: mol_type = other RNA
gctgggattacaggcatgagccatcatgccctgcctgtagttcacttttaagtatattttttaaaagtaaaaaatctgaagcagctgccacccaagtgtagaatagataaattgtgatataatcatagaatgaaaccagacataaccatgaagagaactgaactactgctagacaggacaacgtggatgaatctcacatgcaggatgctgatccggacaccacaagaaaaaacaaaagaaggtgcctactgagttttcttctttccagatgaccaactcttaacttactcatctgtttttttcactgttctgcttcttttgaagaagatttgaggtgacttacaaaggtgtatggcatatttataactgaagaaatctgggtgatgttaaaacgagggcaggaaaataaggtggaaaccagatgtaaggatagtcttcactatttatgtcaggaattcctacaaactttctatggtgaacagaatagagcttcctagcagtcaatgcaaagaagaaacacaacaattccacaccccaaagttaacagtcttgcttatcagaagcacaggtagttctgaaatctgatagaaaatgttcctgtatcatttcagaacacgcaactatgtgatcaaacccctttctatttgtttaaaaatttgtcaaacatcccatgtttgaccctggatgtctgaatcccctcagcccacattttcccccctacaccatgcccacaccatccccatagaatttagggtgaggcagcatctcagtgattgacaggcccctccttagaccccgtttactttcctgggtgtggtttggggtaagccctgttcatgaaggctggatttctgttctttgggttgcccagcttgccaccctcatttctggaacccagaccagcatcctcagcccacgctttgccactcagctcatcttcttcccagttggcacttctcagtgaccccatcccttccccagcagtgactctgcgtggggcagctccctggtggctggactctttccattttggcatttgggttagtggatctttccactttctggctccagtttttgagttgaattcatatgtttccccggtcactggatctatggcttctccatcaaagatagtgttcatctggatagtttccaccacgacgtctctctctgcagtcttcgtttctcctttctttgtcagaggttccttgttcttcccagtcttgcaggggcagtgtctgtggatggctttggccaataggacgaccaggtacacgaggagacccagaagcaatatggagcccaaagtgatgacaaacggcacgtaccatgcagatggagagtaaacgtttttcctcaggacctgataggtgaccctgggcctgggggtcgtggtgatgatagtggttgggtggggaatgactttaatactcagtgtcactgttcctgtctcaacaagagcctccgctttcttcctgtcagacatcaagttgtcatcagttacgtagacaagtagcttgtagtcccagatcttatcaaacccaccagcatagtcaaagcgagatgtaagcagcaggcgtgtgacattggaaccagcattgggagagaaggtgaaatgattgttgacgttaccgggccttctttctgacacatcaaatacataggatggcctatcaaaaatgagaggaaactcattttctgggcttgttaggatataaacgtagacgttatttttatagtaagggggggccacatcctgcacctggattatcaccgtatatttattgccggctgctaggttacttggattttcgtagtctagatcaccaatcagcacaatcttcccagagccagctggatcctgtaaaaatctgctgccgctccccactccagatggcatggtgaagttgaatctgttgtttggtgcctcactgtcatcatcaaagcagaacttgtttaggtcaagaagcaacgtccccttggctgttctttccggcaccataatgctgaaggtgaacttttggcatgtggcaggattgtcgttgacgtcttccacaatgaaggttatctggatgcgattctcctgacccccatatggtctgtccttcactagaacttccagggaaatggtgggattttgtctcaattcacctgcatctcggtctatcctttgggccacttggattgtaccagtcaactgatttatcatgaaatatttgctaacagtggtaatgctgtagaggaggtggctgggaaaaccttcatcatcaggatcctccgctgtgatattggccacgatggttcctggactcagttcctccaggactgtgtacactcgtgtcgggctggtaaagcgagggacttcgtcgttgaggttcacgatgttcacctggagctctgtggaggctttgaggcctccactgtccctcacctccacgatgagatggaaacttctgtgtcctgcttcaaagtccaattctgttgtggagaagagggtgccattagcagacattctgaagctctttgggggagaaatcaggaaataactgaggggaatgtttcggcttgtgtcttctggatcgaaggcctcaacctggtaaatgaatccagggtttgctctttctactatgtagaggtgtagaccttctgccaagttgccttgaaactgaggtggctcgttcacatctgttacctggacagtcaggacttgcaggtctgtgacaccaacctcatccttcacataaatctgcaaatcaaatatgtttggtcctgtttcaaaatctagttgttccatcccagtggtgacaacctgcgtttcagaacgacatctacccactggtttcagctcctagagcaacaactgcagaatctccatggtccaaagtcctccaggaaagagaagaaaggggtgacgggggtgagggctgggaggcgaggtcaccagggtcccttccctggctcgggtgggggtggggggcgcaacccctcacggctcctccccaccaagccgtcgggaccccagcgggggcgcctcgcgttgggcgacagggacgcggggagagagcgacaagctggaagcaagggctgcctgcaaaactttcggtcctccagcggcaactctgcgggaaagaccacccttccttcggccccgcgtcgggcctatccccgtgtgccccgacccctgcgccccaggcttgggcggcgccgctgcatcccggctgccgggcgcgctgcagccttcgctctcccgcacgcggcgctcgcccgtccgcgctgcccctccccggcaggcgggcggccccggcgggcgggcgggc

SEQ ID NO: 15934 - RNA, 3219 nt, Homo sapiens
  source 1..3219: mol_type = other RNA
gctgggattacaggcatgagccatcatgccctgcctgtagttcacttttaagtatattttttaaaagtaaaaaatctgaagcagctgccacccaagtgtagaatagataaattgtgatataatcatagaatgaaaccagacataaccatgaagagaactgaactactgctagacaggacaacgtggatgaatctcacatgcaggatgctgatccggacaccacaagaaaaaacaaaagaaggtgcctactgagttttcttctttccagatgaccaactcttaacttactcatctgtttttttcactgttctgcttcttttgaagaagatttgaggtgacttacaaaggtgtatggcatatttataactgaagaaatctgggtgatgttaaaacgagggcaggaaaataaggtggaaaccagatgtaaggatagtcttcactatttatgtcaggaattcctacaaactttctatggtgaacagaatagagcttcctagcagtcaatgcaaagaagaaacacaacaattccacaccccaaagttaacagtcttgcttatcagaagcacaggtagttctgaaatctgatagaaaatgttcctgtatcatttcagaacacgcaactatgtgatcaaacccctttctatttgtttaaaaatttgtcaaacatcccatgtttgaccctggatgtctgaatcccctcagcccacattttcccccctacaccatgcccacaccatccccatagaatttagggtgaggcagcatctcagtgattgacaggcccctccttagaccccgtttactttcctgggtgtggtttggggtaagccctgttcatgaaggctggatttctgttctttgggttgcccagcttgccaccctcatttctggaacccagaccagcatcctcagcccacgctttgccactcagctcatcttcttcccagttggcacttctcagtgaccccatcccttccccagcagtgactctgcgtggggcagctccctggtggctggactctttccattttggcatttgggttagtggatctttccactttctggctccagtttttgagttgaattcatatgtttccccggtcactggatctatggcttctccatcaaagatagtgttcatctggatagtttccaccacgacgtctctctctgcagtcttcgtttctcctttctttgtcagaggttccttgttcttcccagtcttgcaggggcagtgtctgtggatggctttggccaataggacgaccaggtacacgaggagacccagaagcaatatggagcccaaagtgatgacaaacggcacgtaccatgcagatggagagtaaacgtttttcctcaggacctgataggtgaccctgggcctgggggtcgtggtgatgatagtggttgggtggggaatgactttaatactcagtgtcactgttcctgtctcaacaagagcctccgctttcttcctgtcagacatcaagttgtcatcagttacgtagacaagtagcttgtagtcccagatcttatcaaacccaccagcatagtcaaagcgagatgtaagcagcaggcgtgtgacattggaaccagcattgggagagaaggtgaaatgattgttgacgttaccgggccttctttctgacacatcaaatacataggatggcctatcaaaaatgagaggaaactcattttctgggcttgttaggatataaacgtagacgttatttttatagtaagggggggccacatcctgcacctggattatcaccgtatatttattgccggctgctaggttacttggattttcgtagtctagatcaccaatcagcacaatcttcccagagccagctggatcctgtaaaaatctgctgccgctccccactccagatggcatggtgaagttgaatctgttgtttggtgcctcactgtcatcatcaaagcagaacttgtttaggtcaagaagcaacgtccccttggctgttctttccggcaccataatgctgaaggtgaacttttggcatgtggcaggattgtcgttgacgtcttccacaatgaaggttatctggatgcgattctcctgacccccatatggtctgtccttcactagaacttccagggaaatggtgggattttgtctcaattcacctgcatctcggtctatcctttgggccacttggattgtaccagtcaactgatttatcatgaaatatttgctaacagtggtaatgctgtagaggaggtggctgggaaaaccttcatcatcaggatcctccgctgtgatattggccacgatggttcctggactcagttcctccaggactgtgtacactcgtgtcgggctggtaaagcgagggacttcgtcgttgaggttcacgatgttcacctggagctctgtggaggctttgaggcctccactgtccctcacctccacgatgagatggaaacttctgtgtcctgcttcaaagtccaattctgttgtggagaagagggtgccattagcagacattctgaagctctttgggggagaaatcaggaaatacttctgccaagttgccttgaaactgaggtggctcgttcacatctgttacctggacagtcaggacttgcaggtctgtgacaccaacctcatccttcacataaatctgcaaatcaaatatgtttggtcctgtttcaaaatctagttgttccatcccagtggtgacaacctgcgtttcagaacgacatctacccactggtttcagctcctagagcaacaactgcagaatctccatggtccaaagtcctccaggaaagagaagaaaggggtgacgggggtgagggctgggaggcgaggtcaccagggtcccttccctggctcgggtgggggtggggggcgcaacccctcacggctcctccccaccaagccgtcgggaccccagcgggggcgcctcgcgttgggcgacagggacgcggggagagagcgacaagctggaagcaagggctgcctgcaaaactttcggtcctccagcggcaactctgcgggaaagaccacccttccttcggccccgcgtcgggcctatccccgtgtgccccgacccctgcgccccaggcttgggcggcgccgctgcatcccggctgccgggcgcgctgcagccttcgctctcccgcacgcggcgctcgcccgtccgcgctgcccctccccggcaggcgggcggccccggcgggcgggcgggc

SEQ ID NO: 15935 - RNA, 3019 nt, Homo sapiens
  source 1..3019: mol_type = other RNA
gctgggattacaggcatgagccatcatgccctgcctgtagttcacttttaagtatattttttaaaagtaaaaaatctgaagcagctgccacccaagtgtagaatagataaattgtgatataatcatagaatgaaaccagacataaccatgaagagaactgaactactgctagacaggacaacgtggatgaatctcacatgcaggatgctgatccggacaccacaagaaaaaacaaaagaaggtgcctactgagttttcttctttccagatgaccaactcttaacttactcatctgtttttttcactgttctgcttcttttgaagaagatttgaggtgacttacaaaggtgtatggcatatttataactgaagaaatctgggtgatgttaaaacgagggcaggaaaataaggtggaaaccagatgtaaggatagtcttcactatttatgtcaggaattcctacaaactttctatggtgaacagaatagagcttcctagcagtcaatgcaaagaagaaacacaacaattccacaccccaaagttaacagtcttgcttatcagaagcacaggtagttctgaaatctgatagaaaatgttcctgtatcatttcagaacacgcaactatgtgatcaaacccctttctatttgtttaaaaatttgtcaaacatcccatgtttgaccctggatgtctgaatcccctcagcccacattttcccccctacaccatgcccacaccatccccatagaatttagggtgaggcagcatctcagtgattgacaggcccctccttagaccccgtttactttcctgggtgtggtttggggtaagccctgttcatgaaggctggatttctgttctttgggttgcccagcttgccaccctcatttctggaacccagaccagcatcctcagcccacgctttgccactcagctcatcttcttcccagttggcacttctcagtgaccccatcccttccccagcagtgactctgcgtggggcagctccctggtggctggactctttccattttggcatttgggttagtggatctttccactttctggctccagtttttgagttgaattcatatgtttccccggtcactggatctatggcttctccatcaaagatagtgttcatctggatagtttccaccacgacgtctctctctgcagtcttcgtttctcctttctttgtcagaggttccttgttcttcccagtcttgcaggggcagtgtctgtggatggctttggccaataggacgaccaggtacacgaggagacccagaagcaatatggagcccaaagtgatgacaaacggcacgtaccatgcagatggagagtaaacgtttttcctcaggacctgataggtgaccctgggcctgggggtcgtggtgatgatagtggttgggtggggaatgactttaatactcagtgtcactgttcctgtctcaacaagagcctccgctttcttcctgtcagacatcaagttgtcatcagttacgtagacaagtagcttgtagtcccagatcttatcaaacccaccagcatagtcaaagcgagatgtaagcagcaggcgtgtgacattggaaccagcattgggagagaaggtgaaatgattgttgacgttaccgggccttctttctgacacatcaaatacataggatggcctatcaaaaatgagaggaaactcattttctgggcttgttaggatataaacgtagacgttatttttatagtaagggggggccacatcctgcacctggattatcaccgtatatttattgccggctgctaggttacttggattttcgtagtctagatcaccaatcagcacaatcttcccagagccagctggatcctgtaaaaatctgctgccgctccccactccagatggcatggtgaagttgaatctgttgtttggtgcctcactgtcatcatcaaagcagaacttgtttaggtcaagaagcaacgtccccttggctgttctttccggcaccataatgctgaaggtgaacttttggcatgtggcaggattgtcgttgacgtcttccacaatgaaggttatctggatgcgattctcctgacccccatatggtctgtccttcactagaacttccagggaaatggtgggattttgtctcaattcacctgcatctcggtctatcctttgggccacttggattgtaccagtcaactgatttatcatgaaatatttgctaacagtggtaatgctgtagaggaggtggctgggaaaaccttcatcatcaggatcctccgctgtgatattggccacgatggttcctggactcagttcctccaggactgtgtacactcgtgtcgggcttctgccaagttgccttgaaactgaggtggctcgttcacatctgttacctggacagtcaggacttgcaggtctgtgacaccaacctcatccttcacataaatctgcaaatcaaatatgtttggtcctgtttcaaaatctagttgttccatcccagtggtgacaacctgcgtttcagaacgacatctacccactggtttcagctcctagagcaacaactgcagaatctccatggtccaaagtcctccaggaaagagaagaaaggggtgacgggggtgagggctgggaggcgaggtcaccagggtcccttccctggctcgggtgggggtggggggcgcaacccctcacggctcctccccaccaagccgtcgggaccccagcgggggcgcctcgcgttgggcgacagggacgcggggagagagcgacaagctggaagcaagggctgcctgcaaaactttcggtcctccagcggcaactctgcgggaaagaccacccttccttcggccccgcgtcgggcctatccccgtgtgccccgacccctgcgccccaggcttgggcggcgccgctgcatcccggctgccgggcgcgctgcagccttcgctctcccgcacgcggcgctcgcccgtccgcgctgcccctccccggcaggcgggcggccccggcgggcgggcgggc

SEQ ID NO: 15936 - RNA, 6084 nt, Homo sapiens
  source 1..6084: mol_type = other RNA
gctgggattacaggcatgagccatcatgccctgcctgtagttcacttttaagtatattttttaaaagtaaaaaatctgaagcagctgccacccaagtgtagaatagataaattgtgatataatcatagaatgaaaccagacataaccatgaagagaactgaactactgctagacaggacaacgtggatgaatctcacatgcaggatgctgatccggacaccacaagaaaaaacaaaagaaggtgcctactgagttttcttctttccagatgaccaactcttaacttactcatctgtttttttcactgttctgcttcttttgaagaagatttgaggtgacttacaaaggtgtatggcatatttataactgaagaaatctgggtgatgttaaaacgagggcaggaaaataaggtggaaaccagatgtaaggatagtcttcactatttatgtcaggaattcctacaaactttctatggtgaacagaatagagcttcctagcagtcaatgcaaagaagaaacacaacaattccacaccccaaagttaacagtcttgcttatcagaagcacaggtagttctgaaatctgatagaaaatgttcctgtatcatttcagaacacgcaactatgtgatcaaacccctttctatttgtttaaaaatttgtcaaacatcccatgtttgaccctggatgtctgaatcccctcagcccacattttcccccctacaccatgcccacaccatccccatagaatttagggtgaggcagcatctcagtgattgacaggcccctccttagaccccgtttactttcctgggtgtggtttggggtaagccctgttcatgaaggctggatttctgttctttgggttgcccagcttgccaccctcatttctggaacccagaccagcatcctcagcccacgctttgccactcagctcatcttcttcccagttggcacttctcagtgaccccatcccttccccagcagtgactctgcgtggggcagctccctggtggctggactctttccattttggcatttgggttagtggatctttccactttctggctccagtttttgagttgaattcatatgtttccccggtcactggatctatggcttctccatcaaagatagtgttcatctggatagtttccaccacgacgtctctctctgcagtcttcgtttctcctttctttgtcagaggttccttgttcttcccagtcttgcaggggcagtgtctgtggatggctttggccaataggacgaccaggtacacgaggagacccagaagcaatatggagcccaaagtgatgacaaacggcacgtaccatgcagatggagagtaaacgtttttcctcaggacctgataggtgaccctgggcctgggggtcgtggtgatgatagtggttgggtggggaatgactttaatactcagtgtcactgttcctgtctcaacaagagcctccgctttcttcctgtcagacatcaagttgtcatcagttacgtagacaagtagcttgtagtcccagatcttatcaaacccaccagcatagtcaaagcgagatgtaagcagcaggcgtgtgacattggaaccagcattgggagagaaggtgaaatgattgttgacgttacctgggccaatggaataacggaaagatctggggctggaatcaaggtcggtacatgtcagcttgaaattctgaatatttgtgccaactttcagatccactgggagggccaggaaataagagtttggagtacaaattggcttttcatcattttcttcaaggatgttcacagtaacagtgacagagcttgtgtcttcgttgttggtggcctggattctgagaatatagatgggggttgtttcacagtccactttagttaccagctggagttctcctgtcttgggattaatccaaaatacatttggatactggaggctggcccctccagtggagatggagtacaggaggctgctctgggggaggtctttatcagtggctcgcacctgtcccactcgggttctggcgggccttctttctgacacatcaaatacataggatggcctatcaaaaatgagaggaaactcattttctgggcttgttaggatataaacgtagacgttatttttatagtaagggggggccacatcctgcacctggattatcaccgtatatttattgccggctgctaggttacttggattttcgtagtctagatcaccaatcagcacaatcttcccagagccagctggatcctgtaaaaatctgctgccgctccccactccagatggcatggtgaagttgaatctgttgtttggtgcctcactgtcatcatcaaagcagaacttgtttaggtcaagaagcaacgtccccttggctgttctttccggcaccataatgccccaaactcagagccttccgatcaagcccagcttgctgtaggaggctctgaggaagaccaatgaacaccttgagacttccattcattgaggggctttctcatgtctccaggtttcagttcctccatctataaaatggacataaatgatatcaattagtttttactacataacacactgtcccaaaactgagtgaattaaaacaacaagcatttatggtttctcacagtactataggttttcccacagtcctttcggttttagtttggcttagctggtctctgtggtcactgacagcttggctggggctggacagtctaggatggcctcactcacatgcctggtggtgggaaggtgcttgatttctgcttcttcttgtcctcatcttctaggaggctagtctaggctcattgcatggaggtctctggttccaaaagtaacaagagagggcaagtcccaaggcacatgcatttttcaagcctccgttgtgccatgtttgtgaatgctccagtggtcaaagcaattcacgtggtcaagctcagattcaaggagacccatctcttgatggagctaatagcaaaatcacattgcaaaggagcatgcataaagagcaagcagggaggaatttgcggcttttctttcttttttgtttgttttggctacctatcttaatcatattttgccttggtagaatttcttacaaaaatatatcgtggctgtcatgagaatgtgcctggaagacctttaaccatgagagcataactgaccatcggcctcagctgctgggctctgaaatccatcactgtgtttgtggtgaggccacgtaccaacaactggtcatggcaaagatactaaggctcattcctgtcctatgtcagttgacactggctccaggacccccaatgccctagctgaacactccttaactgcatggcagcctagaatatgtccaactaccttttctccctctttccttcactcagatcagccttgcatcatgatctgatgacttgcccagccttgtccatctctctccccattttctgccacaggcatctcccctaataatagccttgcacatttaatcccatcttagcatctggttcttggagcatacacttctctctgcaaccaaactctgttcccttctttgttccacatcctcttttcatggcagataaaatcagctctgggctcagtgcatacggagcaaagtctgacagcaagaatggtcatgggccactgaggataacaggtttgcttgctggagcgtgtaatggagtctccacgatgcctcattggcaaagatcacctctgtatttcagcaggattggagtctgaacattcctgccttgattgcacaatgtcatggtttcattcatagggacttagaagagacaccacttattaaacaccaactgcatgctgtatcataccaagcactttaaaaacactatctctaatttcctcatctcagagaggtttgtattcttgtccccactgcacaggggaagaaagagtggttccgagcattttcaaggcctgtccaggaaagtggatgtatccagacttgatcctctgcagtgttagagtcactgtaaactttaacttccatgcataagtatccaggctcacagatggtttggggatctaagccttgatttcaactctgcagaagccaggagattgcatcatttaaagaatccaaggtcccgaagccagacatttcaggcactccaacagaggcctcctcacttggccctccagggctgcttggcctgttctctcattcgtccctgacagttggtattcttcccctaaacgcctaacttggaaagccactcccctcattcagcaatccctgcctcaaaagcgagctgccctcgctcccagccatcagaccatgtttctctccccatgcaaagttgactgtgtccagcccattctgaatcagccaaactgctccgcctcttgctcacaaacagcttgcaaagcgctttcactgaatcgcctgacaatttacaaccagagcgggggttgtcacgtgcctcggatgcctccgtcgggccctgggctcattcatcatcagcctgggaaagcctcaggggccacggtacgaaaggctgggagcctgcaggagcccgcgcgggcagcagggggcgcccgcctcctccacgccgccctcctccctgcgggagcacagcacaccgcctccagcagccgcgctgacctcacccgctctgccacctgctctcaagaactccacagcagagaccgcgcccacagcctccaaggaaggaacaaacattcaagagcaagtgtcagagactgtggcagaaccatgccattgtcactttgttctgttttgacctgcttgcgtgcttggctttgacatagttggactggagaaggtataaggctgggaggatggcgggtgctgcaggtcagggcttctcagccctctccgcacccgcccttatgcagccttgggacgcgaggctgggctttaggctgaagacctccgcccctggaactgcagaggaggggtccctttcgttgcccttcctcacatcttggcgttcatagggtggctgagagttcctcccgctagaagagcccaaagagggaacttgagccttggttagattatcttcagtaataaatgcagttagtccagctacggatttcacattggccttcagggctaatctggagggaagattatcaagtgcaggactctgtttggtcttgcctggacagtctaggatattcgaattgcagtttcaccagctaatatggaacacagtctgcaaactgtcctcccatactccaggggactctggactgcaggaagccaaatatacaattaacagatatgcactgaagagagaaaatggacaaggaagatttgagacagcacagccctctccaggcattctcacttcttaaccttcaccccctacctcttagggcagaggaacaaggaagagcaggagggcagaagagggcaggagcttcccaggatgtactggaaccacccaagagttctagcacagatttaaaatgtcaaagaaagtgtaagtgtgatgctgcaaattgtctccactccatcccctgggcccagacatctctcaatttatgcacgtaaaggtgtggaagtcacaatcctaactacccatgcagctgtccccacccatctaatggacttgtagggcttaggttgggataggaacctactacatgcttaagattgtgactgacgttattggggtgtcagcaggaagcagctggtgaattaggatcattctaggaggggtcagtaaagggactatgaagaaggtgctcacagagtatatggaaatctcatcagatggtgcaatatctcagggctcgtgagagtgaagcacccttaccaccactaggcccagggaagccagtggaggaagcaggtcctgcgacagagagctgcttttgggaatggagatcttcaggcagggaagggatgcacccagctcacaaagagagagcctgaccctcctctccttctctttccaggactccccattggccaactagaagctggaaggcaagggagttggttggtatctgatatggtttggctgtgtccccacccaaatctcatcttgaactcccacatgttgtgagagggacccagtagg

SEQ ID NO: 15937 - RNA, 2942 nt, Homo sapiens
  source 1..2942: mol_type = other RNA
gctgggattacaggcatgagccatcatgccctgcctgtagttcacttttaagtatattttttaaaagtaaaaaatctgaagcagctgccacccaagtgtagaatagataaattgtgatataatcatagaatgaaaccagacataaccatgaagagaactgaactactgctagacaggacaacgtggatgaatctcacatgcaggatgctgatccggacaccacaagaaaaaacaaaagaaggtgcctactgagttttcttctttccagatgaccaactcttaacttactcatctgtttttttcactgttctgcttcttttgaagaagatttgaggtgacttacaaaggtgtatggcatatttataactgaagaaatctgggtgatgttaaaacgagggcaggaaaataaggtggaaaccagatgtaaggatagtcttcactatttatgtcaggaattcctacaaactttctatggtgaacagaatagagcttcctagcagtcaatgcaaagaagaaacacaacaattccacaccccaaagttaacagtcttgcttatcagaagcacaggtagttctgaaatctgatagaaaatgttcctgtatcatttcagaacacgcaactatgtgatcaaacccctttctatttgtttaaaaatttgtcaaacatcccatgtttgaccctggatgtctgaatcccctcagcccacattttcccccctacaccatgcccacaccatccccatagaatttagggtgaggcagcatctcagtgattgacaggcccctccttagaccccgtttactttcctgggtgtggtttggggtaagccctgttcatgaaggctggatttctgttctttgggttgcccagcttgccaccctcatttctggaacccagaccagcatcctcagcccacgctttgccactcagctcatcttcttcccagttggcacttctcagtgaccccatcccttccccagcagtgactctgcgtggggcagctccctggtggctggactctttccattttggcatttgggttagtggatctttccactttctggctccagtttttgagttgaattcatatgtttccccggtcactggatctatggcttctccatcaaagatagtgttcatctggatagtttccaccacgacgtctctctctgcagtcttcgtttctcctttctttgtcagaggttccttgttcttcccagtcttgcaggggcagtgtctgtggatggctttggccaataggacgaccaggtacacgaggagacccagaagcaatatggagcccaaagtgatgacaaacggcacgtaccatgcagatggagagtaaacgtttttcctcaggacctgataggtgaccctgggcctgggggtcgtggtgatgatagtggttgggtggggaatgactttaatactcagtgtcactgttcctgtctcaacaagagcctccgctttcttcctgtcagacatcaagttgtcatcagttacgtagacaagtagcttgtagtcccagatcttatcaaacccaccagcatagtcaaagcgagatgtaagcagcaggcgtgtgacattggaaccagcattgggagagaaggtgaaatgattgttgacgttacctgggccaatggaataacggaaagatctggggctggaatcaaggtcggtacatgtcagcttgaaattctgaatatttgtgccaactttcagatccactgggagggccaggaaataagagtttggagtacaaattggcttttcatcattttcttcaaggatgttcacagtaacagtgacagagcttgtgtcttcgttgttggtggcctggattctgagaatatagatgggggttgtttcacagtccactttagttaccagctggagttctcctgtcttgggattaatccaaaatacatttggatactggaggctggcccctccagtggagatggagtacaggaggctgctctgggggaggtctttatcagtggctcgcacctgtcccactcgggttctggcgggccttctttctgacacatcaaatacataggatggcctatcaaaaatgagaggaaactcattttctgggcttgttaggatataaacgtagacgttatttttatagtaagggggggccacatcctgcacctggattatcaccgtatatttattgccggctgctaggttacttggattttcgtagtctagatcaccaatcagcacaatcttcccagagccagctggatcctgtaaaaatctgctgccgctccccactccagatggcatggtgaagttgaatctgttgtttggtgcctcactgtcatcatcaaagcagaacttgtttaggtcaagaagcaacgtccccttggctgttctttccggcaccataatgctgaaggtgaacttttggcatgtggcaggattgtcgttgacgtcttccacaatgaaggttatctggatgcgattctcctgacccccatatggtctgtccttcactagaacttccagggaaatggtgggattttgtctcaattcacctgcatctcggtctatcctttgggccacttggattgtaccagtcaactgaggggaatgtttcggcttgtgtcttctggatcgaaggcctcaacctggtaaatgaatccagggtttgctctttctactatgtagaggtgtagaccttctgccaagttgccttgaaactgaggtggctcgttcacatctgttacctggacagtcaggacttgcaggtctgtgacaccaacctcatccttcacataaatctgcaaatcaaatatgtttggtcctgtttcaaaatctagttgttccatcccagtggtgacaacctgacatggcacccaggagagccaggagaatgattgcttcctgcatacttgatggtcacaactgtgcgtgcttccagcacatt

SEQ ID NO: 15938 - RNA, 3512 nt, Homo sapiens
  source 1..3512: mol_type = other RNA
gctgggattacaggcatgagccatcatgccctgcctgtagttcacttttaagtatattttttaaaagtaaaaaatctgaagcagctgccacccaagtgtagaatagataaattgtgatataatcatagaatgaaaccagacataaccatgaagagaactgaactactgctagacaggacaacgtggatgaatctcacatgcaggatgctgatccggacaccacaagaaaaaacaaaagaaggtgcctactgagttttcttctttccagatgaccaactcttaacttactcatctgtttttttcactgttctgcttcttttgaagaagatttgaggtgacttacaaaggtgtatggcatatttataactgaagaaatctgggtgatgttaaaacgagggcaggaaaataaggtggaaaccagatgtaaggatagtcttcactatttatgtcaggaattcctacaaactttctatggtgaacagaatagagcttcctagcagtcaatgcaaagaagaaacacaacaattccacaccccaaagttaacagtcttgcttatcagaagcacaggtagttctgaaatctgatagaaaatgttcctgtatcatttcagaacacgcaactatgtgatcaaacccctttctatttgtttaaaaatttgtcaaacatcccatgtttgaccctggatgtctgaatcccctcagcccacattttcccccctacaccatgcccacaccatccccatagaatttagggtgaggcagcatctcagtgattgacaggcccctccttagaccccgtttactttcctgggtgtggtttggggtaagccctgttcatgaaggctggatttctgttctttgggttgcccagcttgccaccctcatttctggaacccagaccagcatcctcagcccacgctttgccactcagctcatcttcttcccagttggcacttctcagtgaccccatcccttccccagcagtgactctgcgtggggcagctccctggtggctggactctttccattttggcatttgggttagtggatctttccactttctggctccagtttttgagttgaattcatatgtttccccggtcactggatctatggcttctccatcaaagatagtgttcatctggatagtttccaccacgacgtctctctctgcagtcttcgtttctcctttctttgtcagaggttccttgttcttcccagtcttgcaggggcagtgtctgtggatggctttggccaataggacgaccaggtacacgaggagacccagaagcaatatggagcccaaagtgatgacaaacggcacgtaccatgcagatggagagtaaacgtttttcctcaggacctgataggtgaccctgggcctgggggtcgtggtgatgatagtggttgggtggggaatgactttaatactcagtgtcactgttcctgtctcaacaagagcctccgctttcttcctgtcagacatcaagttgtcatcagttacgtagacaagtagcttgtagtcccagatcttatcaaacccaccagcatagtcaaagcgagatgtaagcagcaggcgtgtgacattggaaccagcattgggagagaaggtgaaatgattgttgacgttacctgggccaatggaataacggaaagatctggggctggaatcaaggtcggtacatgtcagcttgaaattctgaatatttgtgccaactttcagatccactgggagggccaggaaataagagtttggagtacaaattggcttttcatcattttcttcaaggatgttcacagtaacagtgacagagcttgtgtcttcgttgttggtggcctggattctgagaatatagatgggggttgtttcacagtccactttagttaccagctggagttctcctgtcttgggattaatccaaaatacatttggatactggaggctggcccctccagtggagatggagtacaggaggctgctctgggggaggtctttatcagtggctcgcacctgtcccactcgggttctggcgggccttctttctgacacatcaaatacataggatggcctatcaaaaatgagaggaaactcattttctgggcttgttaggatataaacgtagacgttatttttatagtaagggggggccacatcctgcacctggattatcaccgtatatttattgccggctgctaggttacttggattttcgtagtctagatcaccaatcagcacaatcttcccagagccagctggatcctgtaaaaatctgctgccgctccccactccagatggcatggtgaagttgaatctgttgtttggtgcctcactgtcatcatcaaagcagaacttgtttaggtcaagaagcaacgtccccttggctgttctttccggcaccataatgctgaaggtgaacttttggcatgtggcaggattgtcgttgacgtcttccacaatgaaggttatctggatgcgattctcctgacccccatatggtctgtccttcactagaacttccagggaaatggtgggattttgtctcaattcacctgcatctcggtctatcctttgggccacttggattgtaccagtcaactgatttatcatgaaatatttgctaacagtggtaatgctgtagaggaggtggctgggaaaaccttcatcatcaggatcctccgctgtgatattggccacgatggttcctggactcagttcctccaggactgtgtacactcgtgtcgggctggtaaagcgagggacttcgtcgttgaggttcacgatgttcacctggagctctgtggaggctttgaggcctccactgtccctcacctccacgatgagatggaaacttctgtgtcctgcttcaaagtccaattctgttgtggagaagagggtgccattagcagacattctgaagctctttgggggagaaatcaggaaataactgaggggaatgtttcggcttgtgtcttctggatcgaaggcctcaacctggtaaatgaatccagggtttgctctttctactatgtagaggtgtagaccttctgccaagttgccttgaaactgaggtggctcgttcacatctgttacctggacagtcaggacttgcaggtctgtgacaccaacctcatccttcacataaatctgcaaatcaaatatgtttggtcctgtttcaaaatctagttgttccatcccagtggtgacaacctcaaagtaggtgcctgacagccaattcaccctaaaagcttcagtgaggggatttgagttgactatctggggaaatcctgggatcacaggtgacaatgatgctgataacttcacagaaaacttgtgcactgaagtcccaggtggagaattctctgccacattgcctgtagcaggtaagaggattaggtgtagtgcttctccccctgacatggcacccaggagagccaggagaatgattgcttcctgcatacttgatggtcacaactgtgcgtgcttccagcacattagccacagcctgaatccc

SEQ ID NO: 15939 - RNA, 3309 nt, Homo sapiens
  source 1..3309: mol_type = other RNA
gctgggattacaggcatgagccatcatgccctgcctgtagttcacttttaagtatattttttaaaagtaaaaaatctgaagcagctgccacccaagtgtagaatagataaattgtgatataatcatagaatgaaaccagacataaccatgaagagaactgaactactgctagacaggacaacgtggatgaatctcacatgcaggatgctgatccggacaccacaagaaaaaacaaaagaaggtgcctactgagttttcttctttccagatgaccaactcttaacttactcatctgtttttttcactgttctgcttcttttgaagaagatttgaggtgacttacaaaggtgtatggcatatttataactgaagaaatctgggtgatgttaaaacgagggcaggaaaataaggtggaaaccagatgtaaggatagtcttcactatttatgtcaggaattcctacaaactttctatggtgaacagaatagagcttcctagcagtcaatgcaaagaagaaacacaacaattccacaccccaaagttaacagtcttgcttatcagaagcacaggtagttctgaaatctgatagaaaatgttcctgtatcatttcagaacacgcaactatgtgatcaaacccctttctatttgtttaaaaatttgtcaaacatcccatgtttgaccctggatgtctgaatcccctcagcccacattttcccccctacaccatgcccacaccatccccatagaatttagggtgaggcagcatctcagtgattgacaggcccctccttagaccccgtttactttcctgggtgtggtttggggtaagccctgttcatgaaggctggatttctgttctttgggttgcccagcttgccaccctcatttctggaacccagaccagcatcctcagcccacgctttgccactcagctcatcttcttcccagttggcacttctcagtgaccccatcccttccccagcagtgactctgcgtggggcagctccctggtggctggactctttccattttggcatttgggttagtggatctttccactttctggctccagtttttgagttgaattcatatgtttccccggtcactggatctatggcttctccatcaaagatagtgttcatctggatagtttccaccacgacgtctctctctgcagtcttcgtttctcctttctttgtcagaggttccttgttcttcccagtcttgcaggggcagtgtctgtggatggctttggccaataggacgaccaggtacacgaggagacccagaagcaatatggagcccaaagtgatgacaaacggcacgtaccatgcagatggagagtaaacgtttttcctcaggacctgataggtgaccctgggcctgggggtcgtggtgatgatagtggttgggtggggaatgactttaatactcagtgtcactgttcctgtctcaacaagagcctccgctttcttcctgtcagacatcaagttgtcatcagttacgtagacaagtagcttgtagtcccagatcttatcaaacccaccagcatagtcaaagcgagatgtaagcagcaggcgtgtgacattggaaccagcattgggagagaaggtgaaatgattgttgacgttacctgggccaatggaataacggaaagatctggggctggaatcaaggtcggtacatgtcagcttgaaattctgaatatttgtgccaactttcagatccactgggagggccaggaaataagagtttggagtacaaattggcttttcatcattttcttcaaggatgttcacagtaacagtgacagagcttgtgtcttcgttgttggtggcctggattctgagaatatagatgggggttgtttcacagtccactttagttaccagctggagttctcctgtcttgggattaatccaaaatacatttggatactggaggctggcccctccagtggagatggagtacaggaggctgctctgggggaggtctttatcagtggctcgcacctgtcccactcgggttctggcgggccttctttctgacacatcaaatacataggatggcctatcaaaaatgagaggaaactcattttctgggcttgttaggatataaacgtagacgttatttttatagtaagggggggccacatcctgcacctggattatcaccgtatatttattgccggctgctaggttacttggattttcgtagtctagatcaccaatcagcacaatcttcccagagccagctggatcctgtaaaaatctgctgccgctccccactccagatggcatggtgaagttgaatctgttgtttggtgcctcactgtcatcatcaaagcagaacttgtttaggtcaagaagcaacgtccccttggctgttctttccggcaccataatgctgaaggtgaacttttggcatgtggcaggattgtcgttgacgtcttccacaatgaaggttatctggatgcgattctcctgacccccatatggtctgtccttcactagaacttccagggaaatggtgggattttgtctcaattcacctgcatctcggtctatcctttgggccacttggattgtaccagtcaactgatttatcatgaaatatttgctaacagtggtaatgctgtagaggaggtggctgggaaaaccttcatcatcaggatcctccgctgtgatattggccacgatggttcctggactcagttcctccaggactgtgtacactcgtgtcgggctggtaaagcgagggacttcgtcgttgaggttcacgatgttcacctggagctctgtggaggctttgaggcctccactgtccctcacctccacgatgagatggaaacttctgtgtcctgcttcaaagtccaattctgttgtggagaagagggtgccattagcagacattctgaagctctttgggggagaaatcaggaaataactgaggggaatgtttcggcttgtgtcttctggatcgaaggcctcaacctggtaaatgaatccagggtttgctctttctactatgtagaggtgtagaccttctgccaagttgccttgaaactgaggtggctcgttcacatctgttacctggacagtcaggacttgcaggtctgtgacaccaacctcatccttcacataaatctgcaaatcaaatatgtttggtcctgtttcaaaatctagttgttccatcccagtggtgacaacctgacatggcacccaggagagccaggagaatgattgcttcctgcatacttgatggtcacaactgtgcgtgcttccagcacattagccacagcctgaatccc

SEQ ID NO: 15940 - RNA, 3716 nt, Homo sapiens
  source 1..3716: mol_type = other RNA
gctgggattacaggcatgagccatcatgccctgcctgtagttcacttttaagtatattttttaaaagtaaaaaatctgaagcagctgccacccaagtgtagaatagataaattgtgatataatcatagaatgaaaccagacataaccatgaagagaactgaactactgctagacaggacaacgtggatgaatctcacatgcaggatgctgatccggacaccacaagaaaaaacaaaagaaggtgcctactgagttttcttctttccagatgaccaactcttaacttactcatctgtttttttcactgttctgcttcttttgaagaagatttgaggtgacttacaaaggtgtatggcatatttataactgaagaaatctgggtgatgttaaaacgagggcaggaaaataaggtggaaaccagatgtaaggatagtcttcactatttatgtcaggaattcctacaaactttctatggtgaacagaatagagcttcctagcagtcaatgcaaagaagaaacacaacaattccacaccccaaagttaacagtcttgcttatcagaagcacaggtagttctgaaatctgatagaaaatgttcctgtatcatttcagaacacgcaactatgtgatcaaacccctttctatttgtttaaaaatttgtcaaacatcccatgtttgaccctggatgtctgaatcccctcagcccacattttcccccctacaccatgcccacaccatccccatagaatttagggtgaggcagcatctcagtgattgacaggcccctccttagaccccgtttactttcctgggtgtggtttggggtaagccctgttcatgaaggctggatttctgttctttgggttgcccagcttgccaccctcatttctggaacccagaccagcatcctcagcccacgctttgccactcagctcatcttcttcccagttggcacttctcagtgaccccatcccttccccagcagtgactctgcgtggggcagctccctggtggctggactctttccattttggcatttgggttagtggatctttccactttctggctccagtttttgagttgaattcatatgtttccccggtcactggatctatggcttctccatcaaagatagtgttcatctggatagtttccaccacgacgtctctctctgcagtcttcgtttctcctttctttgtcagaggttccttgttcttcccagtcttgcaggggcagtgtctgtggatggctttggccaataggacgaccaggtacacgaggagacccagaagcaatatggagcccaaagtgatgacaaacggcacgtaccatgcagatggagagtaaacgtttttcctcaggacctgataggtgaccctgggcctgggggtcgtggtgatgatagtggttgggtggggaatgactttaatactcagtgtcactgttcctgtctcaacaagagcctccgctttcttcctgtcagacatcaagttgtcatcagttacgtagacaagtagcttgtagtcccagatcttatcaaacccaccagcatagtcaaagcgagatgtaagcagcaggcgtgtgacattggaaccagcattgggagagaaggtgaaatgattgttgacgttacctgggccaatggaataacggaaagatctggggctggaatcaaggtcggtacatgtcagcttgaaattctgaatatttgtgccaactttcagatccactgggagggccaggaaataagagtttggagtacaaattggcttttcatcattttcttcaaggatgttcacagtaacagtgacagagcttgtgtcttcgttgttggtggcctggattctgagaatatagatgggggttgtttcacagtccactttagttaccagctggagttctcctgtcttgggattaatccaaaatacatttggatactggaggctggcccctccagtggagatggagtacaggaggctgctctgggggaggtctttatcagtggctcgcacctgtcccactcgggttctggcgggccttctttctgacacatcaaatacataggatggcctatcaaaaatgagaggaaactcattttctgggcttgttaggatataaacgtagacgttatttttatagtaagggggggccacatcctgcacctggattatcaccgtatatttattgccggctgctaggttacttggattttcgtagtctagatcaccaatcagcacaatcttcccagagccagctggatcctgtaaaaatctgctgccgctccccactccagatggcatggtgaagttgaatctgttgtttggtgcctcactgtcatcatcaaagcagaacttgtttaggtcaagaagcaacgtccccttggctgttctttccggcaccataatgctgaaggtgaacttttggcatgtggcaggattgtcgttgacgtcttccacaatgaaggttatctggatgcgattctcctgacccccatatggtctgtccttcactagaacttccagggaaatggtgggattttgtctcaattcacctgcatctcggtctatcctttgggccacttggattgtaccagtcaactgatttatcatgaaatatttgctaacagtggtaatgctgtagaggaggtggctgggaaaaccttcatcatcaggatcctccgctgtgatattggccacgatggttcctggactcagttcctccaggactgtgtacactcgtgtcgggctggtaaagcgagggacttcgtcgttgaggttcacgatgttcacctggagctctgtggaggctttgaggcctccactgtccctcacctccacgatgagatggaaacttctgtgtcctgcttcaaagtccaattctgttgtggagaagagggtgccattagcagacattctgaagctctttgggggagaaatcaggaaataactgaggggaatgtttcggcttgtgtcttctggatcgaaggcctcaacctggtaaatgaatccagggtttgctctttctactatgtagaggtgtagaccttctgccaagttgccttgaaactgaggtggctcgttcacatctgttacctggacagtcaggacttgcaggtctgtgacaccaacctcatccttcacataaatctgcaaatcaaatatgtttggtcctgtttcaaaatctagttgttccatcccagtggtgacaacctgcgtttcagaacgacatctacccactggtttcagctcctagagcaacaactgcagaatctccatggtccaaagtcctccaggaaagagaagaaaggggtgacgggggtgagggctgggaggcgaggtcaccagggtcccttccctggctcgggtgggggtggggggcgcaacccctcacggctcctccccaccaagccgtcgggaccccagcgggggcgcctcgcgttgggcgacagggacgcggggagagagcgacaagctggaagcaagggctgcctgcaaaactttcggtcctccagcggcaactctgcgggaaagaccacccttccttcggccccgcgtcgggcctatccccgtgtgccccgacccctgcgccccaggcttgggcggcgccgctgcatcccggctgccgggcgcgctgcagccttcgctctcccgcacgcggcgctcgcccgtccgcgctgcccctccccggcaggcgggcggccccggcgggcgggcgggc

SEQ ID NO: 15941 - RNA, 3024 nt, Homo sapiens
  source 1..3024: mol_type = other RNA
gctgggattacaggcatgagccatcatgccctgcctgtagttcacttttaagtatattttttaaaagtaaaaaatctgaagcagctgccacccaagtgtagaatagataaattgtgatataatcatagaatgaaaccagacataaccatgaagagaactgaactactgctagacaggacaacgtggatgaatctcacatgcaggatgctgatccggacaccacaagaaaaaacaaaagaaggtgcctactgagttttcttctttccagatgaccaactcttaacttactcatctgtttttttcactgttctgcttcttttgaagaagatttgaggtgacttacaaaggtgtatggcatatttataactgaagaaatctgggtgatgttaaaacgagggcaggaaaataaggtggaaaccagatgtaaggatagtcttcactatttatgtcaggaattcctacaaactttctatggtgaacagaatagagcttcctagcagtcaatgcaaagaagaaacacaacaattccacaccccaaagttaacagtcttgcttatcagaagcacaggtagttctgaaatctgatagaaaatgttcctgtatcatttcagaacacgcaactatgtgatcaaacccctttctatttgtttaaaaatttgtcaaacatcccatgtttgaccctggatgtctgaatcccctcagcccacattttcccccctacaccatgcccacaccatccccatagaatttagggtgaggcagcatctcagtgattgacaggcccctccttagaccccgtttactttcctgggtgtggtttggggtaagccctgttcatgaaggctggatttctgttctttgggttgcccagcttgccaccctcatttctggaacccagaccagcatcctcagcccacgctttgccactcagctcatcttcttcccagttggcacttctcagtgaccccatcccttccccagcagtgactctgcgtggggcagctccctggtggctggactctttccattttggcatttgggttagtggatctttccactttctggctccagtttttgagttgaattcatatgtttccccggtcactggatctatggcttctccatcaaagatagtgttcatctggatagtttccaccacgacgtctctctctgcagtcttcgtttctcctttctttgtcagaggttccttgttcttcccagtcttgcaggggcagtgtctgtggatggctttggccaataggacgaccaggtacacgaggagacccagaagcaatatggagcccaaagtgatgacaaacggcacgtaccatgcagatggagagtaaacgtttttcctcaggacctgataggtgaccctgggcctgggggtcgtggtgatgatagtggttgggtggggaatgactttaatactcagtgtcactgttcctgtctcaacaagagcctccgctttcttcctgtcagacatcaagttgtcatcagttacgtagacaagtagcttgtagtcccagatcttatcaaacccaccagcatagtcaaagcgagatgtaagcagcaggcgtgtgacattggaaccagcattgggagagaaggtgaaatgattgttgacgttacctgggccaatggaataacggaaagatctggggctggaatcaaggtcggtacatgtcagcttgaaattctgaatatttgtgccaactttcagatccactgggagggccaggaaataagagtttggagtacaaattggcttttcatcattttcttcaaggatgttcacagtaacagtgacagagcttgtgtcttcgttgttggtggcctggattctgagaatatagatgggggttgtttcacagtccactttagttaccagctggagttctcctgtcttgggattaatccaaaatacatttggatactggaggctggcccctccagtggagatggagtacaggaggctgctctgggggaggtctttatcagtggctcgcacctgtcccactcgggttctggcgggccttctttctgacacatcaaatacataggatggcctatcaaaaatgagaggaaactcattttctgggcttgttaggatataaacgtagacgttatttttatagtaagggggggccacatcctgcacctggattatcaccgtatatttattgccggctgctaggttacttggattttcgtagtctagatcaccaatcagcacaatcttcccagagccagctggatcctgtaaaaatctgctgccgctccccactccagatggcatggtgaagttgaatctgttgtttggtgcctcactgtcatcatcaaagcagaacttgtttaggtcaagaagcaacgtccccttggctgttctttccggcaccataatgctgaaggtgaacttttggcatgtggcaggattgtcgttgacgtcttccacaatgaaggttatctggatgcgattctcctgacccccatatggtctgtccttcactagaacttccagggaaatggtgggattttgtctcaattcacctgcatctcggtctatcctttgggccacttggattgtaccagtcaactgatttatcatgaaatatttgctaacagtggtaatgctgtagaggaggtggctgggaaaaccttcatcatcaggatcctccgctgtgatattggccacgatggttcctggactcagttcctccaggactgtgtacactcgtgtcgggctggtaaagcgagggacttcgtcgttgaggttcacgatgttcacctggagctctgtggaggctttgaggcctccactgtccctcacctccacgatgagatggaaacttctgtgtcctgcttcaaagtccaattctgttgtggagaagagggtgccattagcagacattctgaagctctttgggggagaaatcaggaaataatgtttatattcatttcttccaaagggctttaaggttagaaggtttcattatttcctgctaggatgagggatgttctatc

SEQ ID NO: 15942 - RNA, 5732 nt, Homo sapiens
  source 1..5732: mol_type = other RNA
gctgggattacaggcatgagccatcatgccctgcctgtagttcacttttaagtatattttttaaaagtaaaaaatctgaagcagctgccacccaagtgtagaatagataaattgtgatataatcatagaatgaaaccagacataaccatgaagagaactgaactactgctagacaggacaacgtggatgaatctcacatgcaggatgctgatccggacaccacaagaaaaaacaaaagaaggtgcctactgagttttcttctttccagatgaccaactcttaacttactcatctgtttttttcactgttctgcttcttttgaagaagatttgaggtgacttacaaaggtgtatggcatatttataactgaagaaatctgggtgatgttaaaacgagggcaggaaaataaggtggaaaccagatgtaaggatagtcttcactatttatgtcaggaattcctacaaactttctatggtgaacagaatagagcttcctagcagtcaatgcaaagaagaaacacaacaattccacaccccaaagttaacagtcttgcttatcagaagcacaggtagttctgaaatctgatagaaaatgttcctgtatcatttcagaacacgcaactatgtgatcaaacccctttctatttgtttaaaaatttgtcaaacatcccatgtttgaccctggatgtctgaatcccctcagcccacattttcccccctacaccatgcccacaccatccccatagaatttagggtgaggcagcatctcagtgattgacaggcccctccttagaccccgtttactttcctgggtgtggtttggggtaagccctgttcatgaaggctggatttctgttctttgggttgcccagcttgccaccctcatttctggaacccagaccagcatcctcagcccacgctttgccactcagctcatcttcttcccagttggcacttctcagtgaccccatcccttccccagcagtgactctgcgtggggcagctccctggtggctggactctttccattttggcatttgggttagtggatctttccactttctggctccagtttttgagttgaattcatatgtttccccggtcactggatctatggcttctccatcaaagatagtgttcatctggatagtttccaccacgacgtctctctctgcagtcttcgtttctcctttctttgtcagaggttccttgttcttcccagtcttgcaggggcagtgtctgtggatggctttggccaataggacgaccaggtacacgaggagacccagaagcaatatggagcccaaagtgatgacaaacggcacgtaccatgcagatggagagtaaacgtttttcctcaggacctgataggtgaccctgggcctgggggtcgtggtgatgatagtggttgggtggggaatgactttaatactcagtgtcactgttcctgtctcaacaagagcctccgctttcttcctgtcagacatcaagttgtcatcagttacgtagacaagtagcttgtagtcccagatcttatcaaacccaccagcatagtcaaagcgagatgtaagcagcaggcgtgtgacattggaaccagcattgggagagaaggtgaaatgattgttgacgttacctgggccaatggaataacggaaagatctggggctggaatcaaggtcggtacatgtcagcttgaaattctgaatatttgtgccaactttcagatccactgggagggccaggaaataagagtttggagtacaaattggcttttcatcattttcttcaaggatgttcacagtaacagtgacagagcttgtgtcttcgttgttggtggcctggattctgagaatatagatgggggttgtttcacagtccactttagttaccagctggagttctcctgtcttgggattaatccaaaatacatttggatactggaggctggcccctccagtggagatggagtacaggaggctgctctgggggaggtctttatcagtggctcgcacctgtcccactcgggttctggcgggccttctttctgacacatcaaatacataggatggcctatcaaaaatgagaggaaactcattttctgggcttgttaggatataaacgtagacgttatttttatagtaagggggggccacatcctgcacctggattatcaccgtatatttattgccggctgctaggttacttggattttcgtagtctagatcaccaatcagcacaatcttcccagagccagctggatcctgtaaaaatctgctgccgctccccactccagatggcatggtgaagttgaatctgttgtttggtgcctcactgtcatcatcaaagcagaacttgtttaggtcaagaagcaacgtccccttggctgttctttccggcaccataatgctgaaggtgaacttttggcatgtggcaggattgtcgttgacgtcttccacaatgaaggttatctggatgcgattctcctgacccccatatggtctgtccttcactagaacttccagggaaatggtgggattttgtctcaattcacctgcatctcggtctatcctttgggccacttggattgtaccagtcaactgatttatcatgaaatatttgctaacagtggtaatgctgtagaggaggtggctgggaaaaccttcatcatcaggatcctccgctgtgatattggccacgatggttcctggactcagttcctccaggactgtgtacactcgtgtcgggctggtaaagcgagggacttcgtcgttgaggttcacgatgttcacctggagctctgtggaggctttgaggcctccactgtccctcacctccacgatgagatggaaacttctgtgtcctgcttcaaagtccaattctgttgtggagaagagggtgccattagcagacattctgaagctctttgggggagaaatcaggaaataccttgattgtgccttggtgtagggagaaaggaaggtgagagggagctggcccagtttccagaaatgtcagctccctggggtacgaggggaacgccacctccaggcttgcttccccactgcagtaggagtcaccgaccaatgattcaacctgtgccactttgcagctatcagttgctttcagtagaaacaaacaacaagaattcagcttcttgtcttttatagaatagagcagtcaactaccaggccaccgcaggctgagtttccagaaggaaagacccttattcggcccacatccagggagtgtcaatggctccacaagccactgagtacatggccccaaacccaccccagagggccagagcactcaggactgtggcaagttacaaatatgttgccacattcctatatttttcaatggaagctgaatattttgtaaaagcctcaattcctctctttgttttcccctattccaccctcgtctcagctcagaggtgggacgtggaggaggaaggaggaagagtgcctagaagaaaaaaaactatcgttaaaaaactacccactgcaagtccttaacgtggctcctgctcgtggttcattgttctgaggatgagctaagtgggttacaggcaagtacttgaatgtttttaagaagagacacgatgacaaatgcaaaatgctattattaatgtaatccttcaccgataaagctgcagatcctatgccctcacattctgtcattctttttccataattggcctgggttctgtgctgcaagattcaggctttgctaatcttaataacaatgatccccatctatttgagagtgtcccaccccacatgcaaacagccagcagtgaccacatatttggagtgggaattgtccagtacctttgctttttccttttatgagcctttgaacaagaacctggagtagaatgaagaatgccttttgctaagacttcaggtggtgactcctgactcctgagttggcaggcagacaccaggggagctgaatgactggggcaggtgggggtgtatggtggggacagggatgctgtcactcagaaaagcaaggggtaggaagccagtggcagaacttgccagaacagagtagaagggaggtgggtcaggagacctgggttctcactggagttacctgacccctcagttccctccctcatccagaaatcaaggactgcccaatggacctgaaagatcccatccagctgggacccttgatagggccaggtctggcatatgatgaccactttatacacaggaaaaccaaaactcacaactggctgccacttcctagagctatgagcaagataaagacagaaagagaaggatggcccctgctgcgctcccaaaagtccaggtagtagctaggttattgctctcttaatttaatcctttgtctgccttggtgaagacaaagcacatttcattttatgcaaaagcccttcctcaatggaaaggccaaaagaaagccccttaatggagaaattgctgtactagatcattttgcctccagctgagagattgattaacatcctgggagtctccaaggaggctcttctgcagtcacggtggccatttccaagcagagggggaagcagagagtgtgggagttgaatgggaggagggtggtctcaaagagcctccttcagaaagtggagaagaggtgggggggtgggtacccaaagaagaaatgccagtaaaaataattattcacatgcagatcatccttctctatgttctgagcccattattaatgcatacctccaagccaagccccggctctacctgcatgcccaccacaacacagaaggtgcccaggaagggggaaccaatgctagatctaagcctgtgcctggccaatgcagtagccactaccctcacgtacgtgtgactatgagcattgaaatgtggctggtctgcacggagatgatctgtaagtgtaaaatgcacactgagtttggacaccgagtatggaaaaagaaggcaaaatatctcattaatcattttatgttgactatgctgaaatattttgagtatactgagttaaataagctattaaaattaatttcatttattttgttttactttcaatgtggctactagaacatttaaaattacatgtgcaggactcatttctggctcacagtatagctttattggacagagccggtccaatattgatcagtgttggtccaaacaatgtaccagcacatgctttttaagtttcactaaaaagaagggagcaaatacaagtggcttccagattagtacctgtttttcattaactgtgatacagtttcactttattaagctggagaagagttgtaagatttgtcattttaaaggggttgaggtttcaaaatgcatcctatagctatttttaaaaatccattattcattctctagttgctgccaccagcagggtgactcgtggaccccaccaggttaagatgacagacacaaaccaagcctaggtcgcttcaggcatgtgctttagtgttttgttaaactctgtccttgtttgttcagtccagtggttcttgaagtacatggtacatcagaatcaccggggaggtttgtattcaaactcagcattctcaggcaatgtccaggaatctgcatttttaaaatcagcctaagtatgttctaatgcctgaacacacttctaaagcctgcaaaacacttataaaccggtgtttccactgggtgtggtggctcatgtctgtaatcctagcactttgggaggccaaggcaggtggatggcttg

SEQ ID NO: 15943 - RNA, 3821 nt, Homo sapiens
  source 1..3821: mol_type = other RNA
gctgggattacaggcatgagccatcatgccctgcctgtagttcacttttaagtatattttttaaaagtaaaaaatctgaagcagctgccacccaagtgtagaatagataaattgtgatataatcatagaatgaaaccagacataaccatgaagagaactgaactactgctagacaggacaacgtggatgaatctcacatgcaggatgctgatccggacaccacaagaaaaaacaaaagaaggtgcctactgagttttcttctttccagatgaccaactcttaacttactcatctgtttttttcactgttctgcttcttttgaagaagatttgaggtgacttacaaaggtgtatggcatatttataactgaagaaatctgggtgatgttaaaacgagggcaggaaaataaggtggaaaccagatgtaaggatagtcttcactatttatgtcaggaattcctacaaactttctatggtgaacagaatagagcttcctagcagtcaatgcaaagaagaaacacaacaattccacaccccaaagttaacagtcttgcttatcagaagcacaggtagttctgaaatctgatagaaaatgttcctgtatcatttcagaacacgcaactatgtgatcaaacccctttctatttgtttaaaaatttgtcaaacatcccatgtttgaccctggatgtctgaatcccctcagcccacattttcccccctacaccatgcccacaccatccccatagaatttagggtgaggcagcatctcagtgattgacaggcccctccttagaccccgtttactttcctgggtgtggtttggggtaagccctgttcatgaaggctggatttctgttctttgggttgcccagcttgccaccctcatttctggaacccagaccagcatcctcagcccacgctttgccactcagctcatcttcttcccagttggcacttctcagtgaccccatcccttccccagcagtgactctgcgtggggcagctccctggtggctggactctttccattttggcatttgggttagtggatctttccactttctggctccagtttttgagttgaattcatatgtttccccggtcactggatctatggcttctccatcaaagatagtgttcatctggatagtttccaccacgacgtctctctctgcagtcttcgtttctcctttctttgtcagaggttccttgttcttcccagtcttgcaggggcagtgtctgtggatggctttggccaataggacgaccaggtacacgaggagacccagaagcaatatggagcccaaagtgatgacaaacggcacgtaccatgcagatggagagtaaacgtttttcctcaggacctgataggtgaccctgggcctgggggtcgtggtgatgatagtggttgggtggggaatgactttaatactcagtgtcactgttcctgtctcaacaagagcctccgctttcttcctgtcagacatcaagttgtcatcagttacgtagacaagtagcttgtagtcccagatcttatcaaacccaccagcatagtcaaagcgagatgtaagcagcaggcgtgtgacattggaaccagcattgggagagaaggtgaaatgattgttgacgttacctgggccaatggaataacggaaagatctggggctggaatcaaggtcggtacatgtcagcttgaaattctgaatatttgtgccaactttcagatccactgggagggccaggaaataagagtttggagtacaaattggcttttcatcattttcttcaaggatgttcacagtaacagtgacagagcttgtgtcttcgttgttggtggcctggattctgagaatatagatgggggttgtttcacagtccactttagttaccagctggagttctcctgtcttgggattaatccaaaatacatttggatactggaggctggcccctccagtggagatggagtacaggaggctgctctgggggaggtctttatcagtggctcgcacctgtcccactcgggttctggcgggccttctttctgacacatcaaatacataggatggcctatcaaaaatgagaggaaactcattttctgggcttgttaggatataaacgtagacgttatttttatagtaagggggggccacatcctgcacctggattatcaccgtatatttattgccggctgctaggttacttggattttcgtagtctagatcaccaatcagcacaatcttcccagagccagctggatcctgtaaaaatctgctgccgctccccactccagatggcatggtgaagttgaatctgttgtttggtgcctcactgtcatcatcaaagcagaacttgtttaggtcaagaagcaacgtccccttggctgttctttccggcaccataatgctgaaggtgaacttttggcatgtggcaggattgtcgttgacgtcttccacaatgaaggttatctggatgcgattctcctgacccccatatggtctgtccttcactagaacttccagggaaatggtgggattttgtctcaattcacctgcatctcggtctatcctttgggccacttggattgtaccagtcaactgatttatcatgaaatatttgctaacagtggtaatgctgtagaggaggtggctgggaaaaccttcatcatcaggatcctccgctgtgatattggccacgatggttcctggactcagttcctccaggactgtgtacactcgtgtcgggctggtaaagcgagggacttcgtcgttgaggttcacgatgttcacctggagctctgtggaggctttgaggcctccactgtccctcacctccacgatgagatggaaacttctgtgtcctgcttcaaagtccaattctgttgtggagaagagggtgccattagcagacattctgaagctctttgggggagaaatcaggaaatacttctgccaagttgccttgaaactgaggtggctcgttcacatctgttacctggacagtcaggacttgcaggtctgtgacaccaacctcatccttcacataaatctgcaaatcaaatatgtttggtcctgtttcaaaatctagttgttccatcccagtggtgacaacctcaaagtaggtgcctgacagccaattcaccctaaaagcttcagtgaggggatttgagttgactatctggggaaatcctgggatcacaggtgacaatgatgctgataacttcacagaaaacttgtgcactgaagtcccaggtggagaattctctgccacattgcctgtagcaggtaagaggattaggtgtagtgcttctccccctgcgtttcagaacgacatctacccactggtttcagctcctagagcaacaactgcagaatctccatggtccaaagtcctccaggaaagagaagaaaggggtgacgggggtgagggctgggaggcgaggtcaccagggtcccttccctggctcgggtgggggtggggggcgcaacccctcacggctcctccccaccaagccgtcgggaccccagcgggggcgcctcgcgttgggcgacagggacgcggggagagagcgacaagctggaagcaagggctgcctgcaaaactttcggtcctccagcggcaactctgcgggaaagaccacccttccttcggccccgcgtcgggcctatccccgtgtgccccgacccctgcgccccaggcttgggcggcgccgctgcatcccggctgccgggcgcgctgcagccttcgctctcccgcacgcggcgctcgcccgtccgcgctgcccctccccggcaggcgggcggccccggcgggcgggcgggc

SEQ ID NO: 15944 - RNA, 3621 nt, Homo sapiens
  source 1..3621: mol_type = other RNA
gctgggattacaggcatgagccatcatgccctgcctgtagttcacttttaagtatattttttaaaagtaaaaaatctgaagcagctgccacccaagtgtagaatagataaattgtgatataatcatagaatgaaaccagacataaccatgaagagaactgaactactgctagacaggacaacgtggatgaatctcacatgcaggatgctgatccggacaccacaagaaaaaacaaaagaaggtgcctactgagttttcttctttccagatgaccaactcttaacttactcatctgtttttttcactgttctgcttcttttgaagaagatttgaggtgacttacaaaggtgtatggcatatttataactgaagaaatctgggtgatgttaaaacgagggcaggaaaataaggtggaaaccagatgtaaggatagtcttcactatttatgtcaggaattcctacaaactttctatggtgaacagaatagagcttcctagcagtcaatgcaaagaagaaacacaacaattccacaccccaaagttaacagtcttgcttatcagaagcacaggtagttctgaaatctgatagaaaatgttcctgtatcatttcagaacacgcaactatgtgatcaaacccctttctatttgtttaaaaatttgtcaaacatcccatgtttgaccctggatgtctgaatcccctcagcccacattttcccccctacaccatgcccacaccatccccatagaatttagggtgaggcagcatctcagtgattgacaggcccctccttagaccccgtttactttcctgggtgtggtttggggtaagccctgttcatgaaggctggatttctgttctttgggttgcccagcttgccaccctcatttctggaacccagaccagcatcctcagcccacgctttgccactcagctcatcttcttcccagttggcacttctcagtgaccccatcccttccccagcagtgactctgcgtggggcagctccctggtggctggactctttccattttggcatttgggttagtggatctttccactttctggctccagtttttgagttgaattcatatgtttccccggtcactggatctatggcttctccatcaaagatagtgttcatctggatagtttccaccacgacgtctctctctgcagtcttcgtttctcctttctttgtcagaggttccttgttcttcccagtcttgcaggggcagtgtctgtggatggctttggccaataggacgaccaggtacacgaggagacccagaagcaatatggagcccaaagtgatgacaaacggcacgtaccatgcagatggagagtaaacgtttttcctcaggacctgataggtgaccctgggcctgggggtcgtggtgatgatagtggttgggtggggaatgactttaatactcagtgtcactgttcctgtctcaacaagagcctccgctttcttcctgtcagacatcaagttgtcatcagttacgtagacaagtagcttgtagtcccagatcttatcaaacccaccagcatagtcaaagcgagatgtaagcagcaggcgtgtgacattggaaccagcattgggagagaaggtgaaatgattgttgacgttacctgggccaatggaataacggaaagatctggggctggaatcaaggtcggtacatgtcagcttgaaattctgaatatttgtgccaactttcagatccactgggagggccaggaaataagagtttggagtacaaattggcttttcatcattttcttcaaggatgttcacagtaacagtgacagagcttgtgtcttcgttgttggtggcctggattctgagaatatagatgggggttgtttcacagtccactttagttaccagctggagttctcctgtcttgggattaatccaaaatacatttggatactggaggctggcccctccagtggagatggagtacaggaggctgctctgggggaggtctttatcagtggctcgcacctgtcccactcgggttctggcgggccttctttctgacacatcaaatacataggatggcctatcaaaaatgagaggaaactcattttctgggcttgttaggatataaacgtagacgttatttttatagtaagggggggccacatcctgcacctggattatcaccgtatatttattgccggctgctaggttacttggattttcgtagtctagatcaccaatcagcacaatcttcccagagccagctggatcctgtaaaaatctgctgccgctccccactccagatggcatggtgaagttgaatctgttgtttggtgcctcactgtcatcatcaaagcagaacttgtttaggtcaagaagcaacgtccccttggctgttctttccggcaccataatgctgaaggtgaacttttggcatgtggcaggattgtcgttgacgtcttccacaatgaaggttatctggatgcgattctcctgacccccatatggtctgtccttcactagaacttccagggaaatggtgggattttgtctcaattcacctgcatctcggtctatcctttgggccacttggattgtaccagtcaactgatttatcatgaaatatttgctaacagtggtaatgctgtagaggaggtggctgggaaaaccttcatcatcaggatcctccgctgtgatattggccacgatggttcctggactcagttcctccaggactgtgtacactcgtgtcgggcttctgccaagttgccttgaaactgaggtggctcgttcacatctgttacctggacagtcaggacttgcaggtctgtgacaccaacctcatccttcacataaatctgcaaatcaaatatgtttggtcctgtttcaaaatctagttgttccatcccagtggtgacaacctcaaagtaggtgcctgacagccaattcaccctaaaagcttcagtgaggggatttgagttgactatctggggaaatcctgggatcacaggtgacaatgatgctgataacttcacagaaaacttgtgcactgaagtcccaggtggagaattctctgccacattgcctgtagcaggtaagaggattaggtgtagtgcttctccccctgcgtttcagaacgacatctacccactggtttcagctcctagagcaacaactgcagaatctccatggtccaaagtcctccaggaaagagaagaaaggggtgacgggggtgagggctgggaggcgaggtcaccagggtcccttccctggctcgggtgggggtggggggcgcaacccctcacggctcctccccaccaagccgtcgggaccccagcgggggcgcctcgcgttgggcgacagggacgcggggagagagcgacaagctggaagcaagggctgcctgcaaaactttcggtcctccagcggcaactctgcgggaaagaccacccttccttcggccccgcgtcgggcctatccccgtgtgccccgacccctgcgccccaggcttgggcggcgccgctgcatcccggctgccgggcgcgctgcagccttcgctctcccgcacgcggcgctcgcccgtccgcgctgcccctccccggcaggcgggcggccccggcgggcgggcgggc

SEQ ID NO: 15945 - RNA, 3550 nt, Homo sapiens
  source 1..3550: mol_type = other RNA
gctgggattacaggcatgagccatcatgccctgcctgtagttcacttttaagtatattttttaaaagtaaaaaatctgaagcagctgccacccaagtgtagaatagataaattgtgatataatcatagaatgaaaccagacataaccatgaagagaactgaactactgctagacaggacaacgtggatgaatctcacatgcaggatgctgatccggacaccacaagaaaaaacaaaagaaggtgcctactgagttttcttctttccagatgaccaactcttaacttactcatctgtttttttcactgttctgcttcttttgaagaagatttgaggtgacttacaaaggtgtatggcatatttataactgaagaaatctgggtgatgttaaaacgagggcaggaaaataaggtggaaaccagatgtaaggatagtcttcactatttatgtcaggaattcctacaaactttctatggtgaacagaatagagcttcctagcagtcaatgcaaagaagaaacacaacaattccacaccccaaagttaacagtcttgcttatcagaagcacaggtagttctgaaatctgatagaaaatgttcctgtatcatttcagaacacgcaactatgtgatcaaacccctttctatttgtttaaaaatttgtcaaacatcccatgtttgaccctggatgtctgaatcccctcagcccacattttcccccctacaccatgcccacaccatccccatagaatttagggtgaggcagcatctcagtgattgacaggcccctccttagaccccgtttactttcctgggtgtggtttggggtaagccctgttcatgaaggctggatttctgttctttgggttgcccagcttgccaccctcatttctggaacccagaccagcatcctcagcccacgctttgccactcagctcatcttcttcccagttggcacttctcagtgaccccatcccttccccagcagtgactctgcgtggggcagctccctggtggctggactctttccattttggcatttgggttagtggatctttccactttctggctccagtttttgagttgaattcatatgtttccccggtcactggatctatggcttctccatcaaagatagtgttcatctggatagtttccaccacgacgtctctctctgcagtcttcgtttctcctttctttgtcagaggttccttgttcttcccagtcttgcaggggcagtgtctgtggatggctttggccaataggacgaccaggtacacgaggagacccagaagcaatatggagcccaaagtgatgacaaacggcacgtaccatgcagatggagagtaaacgtttttcctcaggacctgataggtgaccctgggcctgggggtcgtggtgatgatagtggttgggtggggaatgactttaatactcagtgtcactgttcctgtctcaacaagagcctccgctttcttcctgtcagacatcaagttgtcatcagttacgtagacaagtagcttgtagtcccagatcttatcaaacccaccagcatagtcaaagcgagatgtaagcagcaggcgtgtgacattggaaccagcattgggagagaaggtgaaatgattgttgacgttacctgggccaatggaataacggaaagatctggggctggaatcaaggtcggtacatgtcagcttgaaattctgaatatttgtgccaactttcagatccactgggagggccaggaaataagagtttggagtacaaattggcttttcatcattttcttcaaggatgttcacagtaacagtgacagagcttgtgtcttcgttgttggtggcctggattctgagaatatagatgggggttgtttcacagtccactttagttaccagctggagttctcctgtcttgggattaatccaaaatacatttggatactggaggctggcccctccagtggagatggagtacaggaggctgctctgggggaggtctttatcagtggctcgcacctgtcccactcgggttctggctggaggaataaagtaccgggccttctttctgacacatcaaatacataggatggcctatcaaaaatgagaggaaactcattttctgggcttgttaggatataaacgtagacgttatttttatagtaagggggggccacatcctgcacctggattatcaccgtatatttattgccggctgctaggttacttggattttcgtagtctagatcaccaatcagcacaatcttcccagagccagctggatcctgtaaaaatctgctgccgctccccactccagatggcatggtgaagttgaatctgttgtttggtgcctcactgtcatcatcaaagcagaacttgtttaggtcaagaagcaacgtccccttggctgttctttccggcaccataatgctgaaggtgaacttttggcatgtggcaggattgtcgttgacgtcttccacaatgaaggttatctggatgcgattctcctgacccccatatggtctgtccttcactagaacttccagggaaatggtgggattttgtctcaattcacctgcatctcggtctatcctttgggccacttggattgtaccagtcaactgatttatcatgaaatatttgctaacagtggtaatgctgtagaggaggtggctgggaaaaccttcatcatcaggatcctccgctgtgatattggccacgatggttcctggactcagttcctccaggactgtgtacactcgtgtcgggctggtaaagcgagggacttcgtcgttgaggttcacgatgttcacctggagctctgtggaggctttgaggcctccactgtccctcacctccacgatgagatggaaacttctgtgtcctgcttcaaagtccaattctgttgtggagaagagggtgccattagcagacattctgaagctctttgggggagaaatcaggaaataactgaggggaatgtttcggcttgtgtcttctggatcgaaggcctcaacctggtaaatgaatccagggtttgctctttctactatgtagaggtgtagaccttctgccaagttgccttgaaactgaggtggctcgttcacatctgttacctggacagtcaggacttgcaggtctgtgacaccaacctcatccttcacataaatctgcaaatcaaatatgtttggtcctgtttcaaaatctagttgttccatcccagtggtgacaacctcaaagtaggtgcctgacagccaattcaccctaaaagcttcagtgaggggatttgagttgactatctggggaaatcctgggatcacaggtgacaatgatgctgataacttcacagaaaacttgtgcactgaagtcccaggtggagaattctctgccacattgcctgtagcaggtaagaggattaggtgtagtgcttctccccctgacatggcacccaggagagccaggagaatgattgcttcctgcatacttgatggtcacaactgtgcgtgcttccagcacattagccacagcctgaatcccgtctcacacccaaagtttatt

SEQ ID NO: 15946 - RNA, 3306 nt, Homo sapiens
  source 1..3306: mol_type = other RNA
gctgggattacaggcatgagccatcatgccctgcctgtagttcacttttaagtatattttttaaaagtaaaaaatctgaagcagctgccacccaagtgtagaatagataaattgtgatataatcatagaatgaaaccagacataaccatgaagagaactgaactactgctagacaggacaacgtggatgaatctcacatgcaggatgctgatccggacaccacaagaaaaaacaaaagaaggtgcctactgagttttcttctttccagatgaccaactcttaacttactcatctgtttttttcactgttctgcttcttttgaagaagatttgaggtgacttacaaaggtgtatggcatatttataactgaagaaatctgggtgatgttaaaacgagggcaggaaaataaggtggaaaccagatgtaaggatagtcttcactatttatgtcaggaattcctacaaactttctatggtgaacagaatagagcttcctagcagtcaatgcaaagaagaaacacaacaattccacaccccaaagttaacagtcttgcttatcagaagcacaggtagttctgaaatctgatagaaaatgttcctgtatcatttcagaacacgcaactatgtgatcaaacccctttctatttgtttaaaaatttgtcaaacatcccatgtttgaccctggatgtctgaatcccctcagcccacattttcccccctacaccatgcccacaccatccccatagaatttagggtgaggcagcatctcagtgattgacaggcccctccttagaccccgtttactttcctgggtgtggtttggggtaagccctgttcatgaaggctggatttctgttctttgggttgcccagcttgccaccctcatttctggaacccagaccagcatcctcagcccacgctttgccactcagctcatcttcttcccagttggcacttctcagtgaccccatcccttccccagcagtgactctgcgtggggcagctccctggtggctggactctttccattttggcatttgggttagtggatctttccactttctggctccagtttttgagttgaattcatatgtttccccggtcactggatctatggcttctccatcaaagatagtgttcatctggatagtttccaccacgacgtctctctctgcagtcttcgtttctcctttctttgtcagaggttccttgttcttcccagtcttgcaggggcagtgtctgtggatggctttggccaataggacgaccaggtacacgaggagacccagaagcaatatggagcccaaagtgatgacaaacggcacgtaccatgcagatggagagtaaacgtttttcctcaggacctgataggtgaccctgggcctgggggtcgtggtgatgatagtggttgggtggggaatgactttaatactcagtgtcactgttcctgtctcaacaagagcctccgctttcttcctgtcagacatcaagttgtcatcagttacgtagacaagtagcttgtagtcccagatcttatcaaacccaccagcatagtcaaagcgagatgtaagcagcaggcgtgtgacattggaaccagcattgggagagaaggtgaaatgattgttgacgttacctgggccaatggaataacggaaagatctggggctggaatcaaggtcggtacatgtcagcttgaaattctgaatatttgtgccaactttcagatccactgggagggccaggaaataagagtttggagtacaaattggcttttcatcattttcttcaaggatgttcacagtaaccgggccttctttctgacacatcaaatacataggatggcctatcaaaaatgagaggaaactcattttctgggcttgttaggatataaacgtagacgttatttttatagtaagggggggccacatcctgcacctggattatcaccgtatatttattgccggctgctaggttacttggattttcgtagtctagatcaccaatcagcacaatcttcccagagccagctggatcctgtaaaaatctgctgccgctccccactccagatggcatggtgaagttgaatctgttgtttggtgcctcactgtcatcatcaaagcagaacttgtttaggtcaagaagcaacgtccccttggctgttctttccggcaccataatgctgaaggtgaacttttggcatgtggcaggattgtcgttgacgtcttccacaatgaaggttatctggatgcgattctcctgacccccatatggtctgtccttcactagaacttccagggaaatggtgggattttgtctcaattcacctgcatctcggtctatcctttgggccacttggattgtaccagtcaactgatttatcatgaaatatttgctaacagtggtaatgctgtagaggaggtggctgggaaaaccttcatcatcaggatcctccgctgtgatattggccacgatggttcctggactcagttcctccaggactgtgtacactcgtgtcgggctggtaaagcgagggacttcgtcgttgaggttcacgatgttcacctggagctctgtggaggctttgaggcctccactgtccctcacctccacgatgagatggaaacttctgtgtcctgcttcaaagtccaattctgttgtggagaagagggtgccattagcagacattctgaagctctttgggggagaaatcaggaaataactgaggggaatgtttcggcttgtgtcttctggatcgaaggcctcaacctggtaaatgaatccagggtttgctctttctactatgtagaggtgtagaccttctgccaagttgccttgaaactgaggtggctcgttcacatctgttacctggacagtcaggacttgcaggtctgtgacaccaacctcatccttcacataaatctgcaaatcaaatatgtttggtcctgtttcaaaatctagttgttccatcccagtggtgacaacctcaaagtaggtgcctgacagccaattcaccctaaaagcttcagtgaggggatttgagttgactatctggggaaatcctgggatcacaggtgacaatgatgctgataacttcacagaaaacttgtgcactgaagtcccaggtggagaattctctgccacattgcctgtagcaggtaagaggattaggtgtagtgcttctccccctgacatggcacccaggagagccaggagaatgattgcttcctgcatacttgatggtcacaactgtgcgtgcttccagcacattagccacagcctgaatcccgtctcacacccaaagtttatt

SEQ ID NO: 15947 - RNA, 3634 nt, Homo sapiens
  source 1..3634: mol_type = other RNA
gctgggattacaggcatgagccatcatgccctgcctgtagttcacttttaagtatattttttaaaagtaaaaaatctgaagcagctgccacccaagtgtagaatagataaattgtgatataatcatagaatgaaaccagacataaccatgaagagaactgaactactgctagacaggacaacgtggatgaatctcacatgcaggatgctgatccggacaccacaagaaaaaacaaaagaaggtgcctactgagttttcttctttccagatgaccaactcttaacttactcatctgtttttttcactgttctgcttcttttgaagaagatttgaggtgacttacaaaggtgtatggcatatttataactgaagaaatctgggtgatgttaaaacgagggcaggaaaataaggtggaaaccagatgtaaggatagtcttcactatttatgtcaggaattcctacaaactttctatggtgaacagaatagagcttcctagcagtcaatgcaaagaagaaacacaacaattccacaccccaaagttaacagtcttgcttatcagaagcacaggtagttctgaaatctgatagaaaatgttcctgtatcatttcagaacacgcaactatgtgatcaaacccctttctatttgtttaaaaatttgtcaaacatcccatgtttgaccctggatgtctgaatcccctcagcccacattttcccccctacaccatgcccacaccatccccatagaatttagggtgaggcagcatctcagtgattgacaggcccctccttagaccccgtttactttcctgggtgtggtttggggtaagccctgttcatgaaggctggatttctgttctttgggttgcccagcttgccaccctcatttctggaacccagaccagcatcctcagcccacgctttgccactcagctcatcttcttcccagttggcacttctcagtgaccccatcccttccccagcagtgactctgcgtggggcagctccctggtggctggactctttccattttggcatttgggttagtggatctttccactttctggctccagtttttgagttgaattcatatgtttccccggtcactggatctatggcttctccatcaaagatagtgttcatctggatagtttccaccacgacgtctctctctgcagtcttcgtttctcctttctttgtcagaggttccttgttcttcccagtcttgcaggggcagtgtctgtggatggctttggccaataggacgaccaggtacacgaggagacccagaagcaatatggagcccaaagtgatgacaaacggcacgtaccatgcagatggagagtaaacgtttttcctcaggacctgataggtgaccctgggcctgggggtcgtggtgatgatagtggttgggtggggaatgactttaatactcagtgtcactgttcctgtctcaacaagagcctccgctttcttcctgtcagacatcaagttgtcatcagttacgtagacaagtagcttgtagtcccagatcttatcaaacccaccagcatagtcaaagcgagatgtaagcagcaggcgtgtgacattggaaccagcattgggagagaaggtgaaatgattgttgacgttacctgggccaatggaataacggaaagatctggggctggaatcaaggtcggtacatgtcagcttgaaattctgaatatttgtgccaactttcagatccactgggagggccaggaaataagagtttggagtacaaattggcttttcatcattttcttcaaggatgttcacagtaacctgcagatgacaccgagttgtttttccaggaaggtgtggatttacggtgtctccatgtgccaccttgcctgctgccccttgtaaatggaacttctttaactagtgacagagcttgtgtcttcgttgttggtggcctggattctgagaatatagatgggggttgtttcacagtccactttagttaccagctggagttctcctgtcttgggattaatccaaaatacatttggatactggaggctggcccctccagtggagatggagtacaggaggctgctctgggggaggtctttatcagtggctcgcacctgtcccactcgggttctggcgggccttctttctgacacatcaaatacataggatggcctatcaaaaatgagaggaaactcattttctgggcttgttaggatataaacgtagacgttatttttatagtaagggggggccacatcctgcacctggattatcaccgtatatttattgccggctgctaggttacttggattttcgtagtctagatcaccaatcagcacaatcttcccagagccagctggatcctgtaaaaatctgctgccgctccccactccagatggcatggtgaagttgaatctgttgtttggtgcctcactgtcatcatcaaagcagaacttgtttaggtcaagaagcaacgtccccttggctgttctttccggcaccataatgctgaaggtgaacttttggcatgtggcaggattgtcgttgacgtcttccacaatgaaggttatctggatgcgattctcctgacccccatatggtctgtccttcactagaacttccagggaaatggtgggattttgtctcaattcacctgcatctcggtctatcctttgggccacttggattgtaccagtcaactgatttatcatgaaatatttgctaacagtggtaatgctgtagaggaggtggctgggaaaaccttcatcatcaggatcctccgctgtgatattggccacgatggttcctggactcagttcctccaggactgtgtacactcgtgtcgggctggtaaagcgagggacttcgtcgttgaggttcacgatgttcacctggagctctgtggaggctttgaggcctccactgtccctcacctccacgatgagatggaaacttctgtgtcctgcttcaaagtccaattctgttgtggagaagagggtgccattagcagacattctgaagctctttgggggagaaatcaggaaataactgaggggaatgtttcggcttgtgtcttctggatcgaaggcctcaacctggtaaatgaatccagggtttgctctttctactatgtagaggtgtagaccttctgccaagttgccttgaaactgaggtggctcgttcacatctgttacctggacagtcaggacttgcaggtctgtgacaccaacctcatccttcacataaatctgcaaatcaaatatgtttggtcctgtttcaaaatctagttgttccatcccagtggtgacaacctcaaagtaggtgcctgacagccaattcaccctaaaagcttcagtgaggggatttgagttgactatctggggaaatcctgggatcacaggtgacaatgatgctgataacttcacagaaaacttgtgcactgaagtcccaggtggagaattctctgccacattgcctgtagcaggtaagaggattaggtgtagtgcttctccccctgacatggcacccaggagagccaggagaatgattgcttcctgcatacttgatggtcacaactgtgcgtgcttccagcacattagccacagcctgaatcccgtctcacacccaaagtttatt

SEQ ID NO: 15948 - RNA, 2883 nt, Homo sapiens
  source 1..2883: mol_type = other RNA
gctgggattacaggcatgagccatcatgccctgcctgtagttcacttttaagtatattttttaaaagtaaaaaatctgaagcagctgccacccaagtgtagaatagataaattgtgatataatcatagaatgaaaccagacataaccatgaagagaactgaactactgctagacaggacaacgtggatgaatctcacatgcaggatgctgatccggacaccacaagaaaaaacaaaagaaggtgcctactgagttttcttctttccagatgaccaactcttaacttactcatctgtttttttcactgttctgcttcttttgaagaagatttgaggtgacttacaaaggtgtatggcatatttataactgaagaaatctgggtgatgttaaaacgagggcaggaaaataaggtggaaaccagatgtaaggatagtcttcactatttatgtcaggaattcctacaaactttctatggtgaacagaatagagcttcctagcagtcaatgcaaagaagaaacacaacaattccacaccccaaagttaacagtcttgcttatcagaagcacaggtagttctgaaatctgatagaaaatgttcctgtatcatttcagaacacgcaactatgtgatcaaacccctttctatttgtttaaaaatttgtcaaacatcccatgtttgaccctggatgtctgaatcccctcagcccacattttcccccctacaccatgcccacaccatccccatagaatttagggtgaggcagcatctcagtgattgacaggcccctccttagaccccgtttactttcctgggtgtggtttggggtaagccctgttcatgaaggctggatttctgttctttgggttgcccagcttgccaccctcatttctggaacccagaccagcatcctcagcccacgctttgccactcagctcatcttcttcccagttggcacttctcagtgaccccatcccttccccagcagtgactctgcgtggggcagctccctggtggctggactctttccattttggcatttgggttagtggatctttccactttctggctccagtttttgagttgaattcatatgtttccccggtcactggatctatggcttctccatcaaagatagtgttcatctggatagtttccaccacgacgtctctctctgcagtcttcgtttctcctttctttgtcagaggttccttgttcttcccagtcttgcaggggcagtgtctgtggatggctttggccaataggacgaccaggtacacgaggagacccagaagcaatatggagcccaaagtgatgacaaacggcacgtaccatgcagatggagagtaaacgtttttcctcaggacctgataggtgaccctgggcgggccttctttctgacacatcaaatacataggatggcctatcaaaaatgagaggaaactcattttctgggcttgttaggatataaacgtagacgttatttttatagtaagggggggccacatcctgcacctggattatcaccgtatatttattgccggctgctaggttacttggattttcgtagtctagatcaccaatcagcacaatcttcccagagccagctggatcctgtaaaaatctgctgccgctccccactccagatggcatggtgaagttgaatctgttgtttggtgcctcactgtcatcatcaaagcagaacttgtttaggtcaagaagcaacgtccccttggctgttctttccggcaccataatgctgaaggtgaacttttggcatgtggcaggattgtcgttgacgtcttccacaatgaaggttatctggatgcgattctcctgacccccatatggtctgtccttcactagaacttccagggaaatggtgggattttgtctcaattcacctgcatctcggtctatcctttgggccacttggattgtaccagtcaactgatttatcatgaaatatttgctaacagtggtaatgctgtagaggaggtggctgggaaaaccttcatcatcaggatcctccgctgtgatattggccacgatggttcctggactcagttcctccaggactgtgtacactcgtgtcgggctggtaaagcgagggacttcgtcgttgaggttcacgatgttcacctggagctctgtggaggctttgaggcctccactgtccctcacctccacgatgagatggaaacttctgtgtcctgcttcaaagtccaattctgttgtggagaagagggtgccattagcagacattctgaagctctttgggggagaaatcaggaaataactgaggggaatgtttcggcttgtgtcttctggatcgaaggcctcaacctggtaaatgaatccagggtttgctctttctactatgtagaggtgtagaccttctgccaagttgccttgaaactgaggtggctcgttcacatctgttacctggacagtcaggacttgcaggtctgtgacaccaacctcatccttcacataaatctgcaaatcaaatatgtttggtcctgtttcaaaatctagttgttccatcccagtggtgacaacctcaaagtaggtgcctgacagccaattcaccctaaaagcttcagtgaggggatttgagttgactatctggggaaatcctgggatcacaggtgacaatgatgctgataacttcacagaaaacttgtgcactgaagtcccaggtggagaattctctgccacattgcctgtagcaggtaagaggattaggtgtagtgcttctccccctgacatggcacccaggagagccaggagaatgattgcttcctgcatacttgatggtcacaactgtgcgtgcttccagcacattagccacagcctgaatcccgtctcacacccaaagtttatt

SEQ ID NO: 15949 - RNA, 3282 nt, Homo sapiens
  source 1..3282: mol_type = other RNA
gctgggattacaggcatgagccatcatgccctgcctgtagttcacttttaagtatattttttaaaagtaaaaaatctgaagcagctgccacccaagtgtagaatagataaattgtgatataatcatagaatgaaaccagacataaccatgaagagaactgaactactgctagacaggacaacgtggatgaatctcacatgcaggatgctgatccggacaccacaagaaaaaacaaaagaaggtgcctactgagttttcttctttccagatgaccaactcttaacttactcatctgtttttttcactgttctgcttcttttgaagaagatttgaggtgacttacaaaggtgtatggcatatttataactgaagaaatctgggtgatgttaaaacgagggcaggaaaataaggtggaaaccagatgtaaggatagtcttcactatttatgtcaggaattcctacaaactttctatggtgaacagaatagagcttcctagcagtcaatgcaaagaagaaacacaacaattccacaccccaaagttaacagtcttgcttatcagaagcacaggtagttctgaaatctgatagaaaatgttcctgtatcatttcagaacacgcaactatgtgatcaaacccctttctatttgtttaaaaatttgtcaaacatcccatgtttgaccctggatgtctgaatcccctcagcccacattttcccccctacaccatgcccacaccatccccatagaatttagggtgaggcagcatctcagtgattgacaggcccctccttagaccccgtttactttcctgggtgtggtttggggtaagccctgttcatgaaggctggatttctgttctttgggttgcccagcttgccaccctcatttctggaacccagaccagcatcctcagcccacgctttgccactcagctcatcttcttcccagttggcacttctcagtgaccccatcccttccccagcagtgactctgcgtggggcagctccctggtggctggactctttccattttggcatttgggttagtggatctttccactttctggctccagtttttgagttgaattcatatgtttccccggtcactggatctatggcttctccatcaaagatagtgttcatctggatagtttccaccacgacgtctctctctgcagtcttcgtttctcctttctttgtcagaggttccttgttcttcccagtcttgcaggggcagtgtctgtggatggctttggccaataggacgaccaggtacacgaggagacccagaagcaatatggagcccaaagtgatgacaaacggcacgtaccatgcagatggagagtaaacgtttttcctcaggacctgataggtgaccctgggctgggccaatggaataacggaaagatctggggctggaatcaaggtcggtacatgtcagcttgaaattctgaatatttgtgccaactttcagatccactgggagggccaggaaataagagtttggagtacaaattggcttttcatcattttcttcaaggatgttcacagtaacagtgacagagcttgtgtcttcgttgttggtggcctggattctgagaatatagatgggggttgtttcacagtccactttagttaccagctggagttctcctgtcttgggattaatccaaaatacatttggatactggaggctggcccctccagtggagatggagtacaggaggctgctctgggggaggtctttatcagtggctcgcacctgtcccactcgggttctggcgggccttctttctgacacatcaaatacataggatggcctatcaaaaatgagaggaaactcattttctgggcttgttaggatataaacgtagacgttatttttatagtaagggggggccacatcctgcacctggattatcaccgtatatttattgccggctgctaggttacttggattttcgtagtctagatcaccaatcagcacaatcttcccagagccagctggatcctgtaaaaatctgctgccgctccccactccagatggcatggtgaagttgaatctgttgtttggtgcctcactgtcatcatcaaagcagaacttgtttaggtcaagaagcaacgtccccttggctgttctttccggcaccataatgctgaaggtgaacttttggcatgtggcaggattgtcgttgacgtcttccacaatgaaggttatctggatgcgattctcctgacccccatatggtctgtccttcactagaacttccagggaaatggtgggattttgtctcaattcacctgcatctcggtctatcctttgggccacttggattgtaccagtcaactgatttatcatgaaatatttgctaacagtggtaatgctgtagaggaggtggctgggaaaaccttcatcatcaggatcctccgctgtgatattggccacgatggttcctggactcagttcctccaggactgtgtacactcgtgtcgggctggtaaagcgagggacttcgtcgttgaggttcacgatgttcacctggagctctgtggaggctttgaggcctccactgtccctcacctccacgatgagatggaaacttctgtgtcctgcttcaaagtccaattctgttgtggagaagagggtgccattagcagacattctgaagctctttgggggagaaatcaggaaataactgaggggaatgtttcggcttgtgtcttctggatcgaaggcctcaacctggtaaatgaatccagggtttgctctttctactatgtagaggtgtagaccttctgccaagttgccttgaaactgaggtggctcgttcacatctgttacctggacagtcaggacttgcaggtctgtgacaccaacctcatccttcacataaatctgcaaatcaaatatgtttggtcctgtttcaaaatctagttgttccatcccagtggtgacaacctcaaagtaggtgcctgacagccaattcaccctaaaagcttcagtgaggggatttgagttgactatctggggaaatcctgggatcacaggtgacaatgatgctgataacttcacagaaaacttgtgcactgaagtcccaggtggagaattctctgccacattgcctgtagcaggtaagaggattaggtgtagtgcttctccccctgacatggcacccaggagagccaggagaatgattgcttcctgcatacttgatggtcacaactgtgcgtgcttccagcacattagccacagcctgaatcccgtctcacacccaaagtttatt

SEQ ID NO: 15950 - RNA, 3299 nt, Homo sapiens
  source 1..3299: mol_type = other RNA
gctgggattacaggcatgagccatcatgccctgcctgtagttcacttttaagtatattttttaaaagtaaaaaatctgaagcagctgccacccaagtgtagaatagataaattgtgatataatcatagaatgaaaccagacataaccatgaagagaactgaactactgctagacaggacaacgtggatgaatctcacatgcaggatgctgatccggacaccacaagaaaaaacaaaagaaggtgcctactgagttttcttctttccagatgaccaactcttaacttactcatctgtttttttcactgttctgcttcttttgaagaagatttgaggtgacttacaaaggtgtatggcatatttataactgaagaaatctgggtgatgttaaaacgagggcaggaaaataaggtggaaaccagatgtaaggatagtcttcactatttatgtcaggaattcctacaaactttctatggtgaacagaatagagcttcctagcagtcaatgcaaagaagaaacacaacaattccacaccccaaagttaacagtcttgcttatcagaagcacaggtagttctgaaatctgatagaaaatgttcctgtatcatttcagaacacgcaactatgtgatcaaacccctttctatttgtttaaaaatttgtcaaacatcccatgtttgaccctggatgtctgaatcccctcagcccacattttcccccctacaccatgcccacaccatccccatagaatttagggtgaggcagcatctcagtgattgacaggcccctccttagaccccgtttactttcctgggtgtggtttggggtaagccctgttcatgaaggctggatttctgttctttgggttgcccagcttgccaccctcatttctggaacccagaccagcatcctcagcccacgctttgccactcagctcatcttcttcccagttggcacttctcagtgaccccatcccttccccagcagtgactctgcgtggggcagctccctggtggctggactctttccattttggcatttgggttagtggatctttccactttctggctccagtttttgagttgaattcatatgtttccccggtcactggatctatggcttctccatcaaagatagtgttcatctggatagtttccaccacgacgtctctctctgcagtcttcgtttctcctttctttgtcagaggttccttgttcttcccagtcttgcaggggcagtgtctgtggatggctttggccaataggacgaccaggtacacgaggagacccagaagcaatatggagcccaaagtgatgacaaacggcacgtaccatgcagatggagagtaaacgtttttcctcaggacctgataggtgaccctgggctgggccaatggaataacggaaagatctggggctggaatcaaggtcggtacatgtcagcttgaaattctgaatatttgtgccaactttcagatccactgggagggccaggaaataagagtttggagtacaaattggcttttcatcattttcttcaaggatgttcacagtaacagtgacagagcttgtgtcttcgttgttggtggcctggattctgagaatatagatgggggttgtttcacagtccactttagttaccagctggagttctcctgtcttgggattaatccaaaatacatttggatactggaggctggcccctccagtggagatggagtacaggaggctgctctgggggaggtctttatcagtggctcgcacctgtcccactcgggttctggctggaggaataaagtaccgggccttctttctgacacatcaaatacataggatggcctatcaaaaatgagaggaaactcattttctgggcttgttaggatataaacgtagacgttatttttatagtaagggggggccacatcctgcacctggattatcaccgtatatttattgccggctgctaggttacttggattttcgtagtctagatcaccaatcagcacaatcttcccagagccagctggatcctgtaaaaatctgctgccgctccccactccagatggcatggtgaagttgaatctgttgtttggtgcctcactgtcatcatcaaagcagaacttgtttaggtcaagaagcaacgtccccttggctgttctttccggcaccataatgctgaaggtgaacttttggcatgtggcaggattgtcgttgacgtcttccacaatgaaggttatctggatgcgattctcctgacccccatatggtctgtccttcactagaacttccagggaaatggtgggattttgtctcaattcacctgcatctcggtctatcctttgggccacttggattgtaccagtcaactgatttatcatgaaatatttgctaacagtggtaatgctgtagaggaggtggctgggaaaaccttcatcatcaggatcctccgctgtgatattggccacgatggttcctggactcagttcctccaggactgtgtacactcgtgtcgggctggtaaagcgagggacttcgtcgttgaggttcacgatgttcacctggagctctgtggaggctttgaggcctccactgtccctcacctccacgatgagatggaaacttctgtgtcctgcttcaaagtccaattctgttgtggagaagagggtgccattagcagacattctgaagctctttgggggagaaatcaggaaataactgaggggaatgtttcggcttgtgtcttctggatcgaaggcctcaacctggtaaatgaatccagggtttgctctttctactatgtagaggtgtagaccttctgccaagttgccttgaaactgaggtggctcgttcacatctgttacctggacagtcaggacttgcaggtctgtgacaccaacctcatccttcacataaatctgcaaatcaaatatgtttggtcctgtttcaaaatctagttgttccatcccagtggtgacaacctcaaagtaggtgcctgacagccaattcaccctaaaagcttcagtgaggggatttgagttgactatctggggaaatcctgggatcacaggtgacaatgatgctgataacttcacagaaaacttgtgcactgaagtcccaggtggagaattctctgccacattgcctgtagcaggtaagaggattaggtgtagtgcttctccccctgacatggcacccaggagagccaggagaatgattgcttcctgcatacttgatggtcacaactgtgcgtgcttccagcacattagccacagcctgaatcccgtctcacacccaaagtttatt

SEQ ID NO: 15951 - RNA, 3055 nt, Homo sapiens
  source 1..3055: mol_type = other RNA
gctgggattacaggcatgagccatcatgccctgcctgtagttcacttttaagtatattttttaaaagtaaaaaatctgaagcagctgccacccaagtgtagaatagataaattgtgatataatcatagaatgaaaccagacataaccatgaagagaactgaactactgctagacaggacaacgtggatgaatctcacatgcaggatgctgatccggacaccacaagaaaaaacaaaagaaggtgcctactgagttttcttctttccagatgaccaactcttaacttactcatctgtttttttcactgttctgcttcttttgaagaagatttgaggtgacttacaaaggtgtatggcatatttataactgaagaaatctgggtgatgttaaaacgagggcaggaaaataaggtggaaaccagatgtaaggatagtcttcactatttatgtcaggaattcctacaaactttctatggtgaacagaatagagcttcctagcagtcaatgcaaagaagaaacacaacaattccacaccccaaagttaacagtcttgcttatcagaagcacaggtagttctgaaatctgatagaaaatgttcctgtatcatttcagaacacgcaactatgtgatcaaacccctttctatttgtttaaaaatttgtcaaacatcccatgtttgaccctggatgtctgaatcccctcagcccacattttcccccctacaccatgcccacaccatccccatagaatttagggtgaggcagcatctcagtgattgacaggcccctccttagaccccgtttactttcctgggtgtggtttggggtaagccctgttcatgaaggctggatttctgttctttgggttgcccagcttgccaccctcatttctggaacccagaccagcatcctcagcccacgctttgccactcagctcatcttcttcccagttggcacttctcagtgaccccatcccttccccagcagtgactctgcgtggggcagctccctggtggctggactctttccattttggcatttgggttagtggatctttccactttctggctccagtttttgagttgaattcatatgtttccccggtcactggatctatggcttctccatcaaagatagtgttcatctggatagtttccaccacgacgtctctctctgcagtcttcgtttctcctttctttgtcagaggttccttgttcttcccagtcttgcaggggcagtgtctgtggatggctttggccaataggacgaccaggtacacgaggagacccagaagcaatatggagcccaaagtgatgacaaacggcacgtaccatgcagatggagagtaaacgtttttcctcaggacctgataggtgaccctgggctgggccaatggaataacggaaagatctggggctggaatcaaggtcggtacatgtcagcttgaaattctgaatatttgtgccaactttcagatccactgggagggccaggaaataagagtttggagtacaaattggcttttcatcattttcttcaaggatgttcacagtaaccgggccttctttctgacacatcaaatacataggatggcctatcaaaaatgagaggaaactcattttctgggcttgttaggatataaacgtagacgttatttttatagtaagggggggccacatcctgcacctggattatcaccgtatatttattgccggctgctaggttacttggattttcgtagtctagatcaccaatcagcacaatcttcccagagccagctggatcctgtaaaaatctgctgccgctccccactccagatggcatggtgaagttgaatctgttgtttggtgcctcactgtcatcatcaaagcagaacttgtttaggtcaagaagcaacgtccccttggctgttctttccggcaccataatgctgaaggtgaacttttggcatgtggcaggattgtcgttgacgtcttccacaatgaaggttatctggatgcgattctcctgacccccatatggtctgtccttcactagaacttccagggaaatggtgggattttgtctcaattcacctgcatctcggtctatcctttgggccacttggattgtaccagtcaactgatttatcatgaaatatttgctaacagtggtaatgctgtagaggaggtggctgggaaaaccttcatcatcaggatcctccgctgtgatattggccacgatggttcctggactcagttcctccaggactgtgtacactcgtgtcgggctggtaaagcgagggacttcgtcgttgaggttcacgatgttcacctggagctctgtggaggctttgaggcctccactgtccctcacctccacgatgagatggaaacttctgtgtcctgcttcaaagtccaattctgttgtggagaagagggtgccattagcagacattctgaagctctttgggggagaaatcaggaaataactgaggggaatgtttcggcttgtgtcttctggatcgaaggcctcaacctggtaaatgaatccagggtttgctctttctactatgtagaggtgtagaccttctgccaagttgccttgaaactgaggtggctcgttcacatctgttacctggacagtcaggacttgcaggtctgtgacaccaacctcatccttcacataaatctgcaaatcaaatatgtttggtcctgtttcaaaatctagttgttccatcccagtggtgacaacctcaaagtaggtgcctgacagccaattcaccctaaaagcttcagtgaggggatttgagttgactatctggggaaatcctgggatcacaggtgacaatgatgctgataacttcacagaaaacttgtgcactgaagtcccaggtggagaattctctgccacattgcctgtagcaggtaagaggattaggtgtagtgcttctccccctgacatggcacccaggagagccaggagaatgattgcttcctgcatacttgatggtcacaactgtgcgtgcttccagcacattagccacagcctgaatcccgtctcacacccaaagtttatt

SEQ ID NO: 15952 - RNA, 3743 nt, Homo sapiens
  source 1..3743: mol_type = other RNA
gctgggattacaggcatgagccatcatgccctgcctgtagttcacttttaagtatattttttaaaagtaaaaaatctgaagcagctgccacccaagtgtagaatagataaattgtgatataatcatagaatgaaaccagacataaccatgaagagaactgaactactgctagacaggacaacgtggatgaatctcacatgcaggatgctgatccggacaccacaagaaaaaacaaaagaaggtgcctactgagttttcttctttccagatgaccaactcttaacttactcatctgtttttttcactgttctgcttcttttgaagaagatttgaggtgacttacaaaggtgtatggcatatttataactgaagaaatctgggtgatgttaaaacgagggcaggaaaataaggtggaaaccagatgtaaggatagtcttcactatttatgtcaggaattcctacaaactttctatggtgaacagaatagagcttcctagcagtcaatgcaaagaagaaacacaacaattccacaccccaaagttaacagtcttgcttatcagaagcacaggtagttctgaaatctgatagaaaatgttcctgtatcatttcagaacacgcaactatgtgatcaaacccctttctatttgtttaaaaatttgtcaaacatcccatgtttgaccctggatgtctgaatcccctcagcccacattttcccccctacaccatgcccacaccatccccatagaatttagggtgaggcagcatctcagtgattgacaggcccctccttagaccccgtttactttcctgggtgtggtttggggtaagccctgttcatgaaggctggatttctgttctttgggttgcccagcttgccaccctcatttctggaacccagaccagcatcctcagcccacgctttgccactcagctcatcttcttcccagttggcacttctcagtgaccccatcccttccccagcagtgactctgcgtggggcagctccctggtggctggactctttccattttggcatttgggttagtggatctttccactttctggctccagtttttgagttgaattcatatgtttccccggtcactggatctatggcttctccatcaaagatagtgttcatctggatagtttccaccacgacgtctctctctgcagtcttcgtttctcctttctttgtcagaggttccttgttcttcccagtcttgcaggggcagtgtctgtggatggctttggccaataggacgaccaggtacacgaggagacccagaagcaatatggagcccaaagtgatgacaaacggcacgtaccatgcagatggagagtaaacgtttttcctcaggacctgataggtgaccctgggctgggccaatggaataacggaaagatctggggctggaatcaaggtcggtacatgtcagcttgaaattctgaatatttgtgccaactttcagatccactgggagggccaggaaataagagtttggagtacaaattggcttttcatcattttcttcaaggatgttcacagtaacctagagtagcaagaaggtggtcattctcaatagctaaaactcattgagtgcttactgtgtgtaggcagttttcaggctaagcacttttcataaattagctcatttaaactcacatgagatagctaacatgattattcccattttatggtgagaaaatggaagtttagagagactaggtaattgatctaagatcattcagctagtgaatggcagagttgggatttgaattcaggtctgtcctactccaaatcctatgctattaacttctacaccatatgcatgtgtgtgtgcacatttagtgtatgtataccttgccccccccccacacacacacacatgcacctggacacataggctcacctgcagatgacaccgagttgtttttccaggaaggtgtggatttacggtgtctccatgtgccaccttgcctgctgccccttgtaaatggaacttctttaactagtgacagagcttgtgtcttcgttgttggtggcctggattctgagaatatagatgggggttgtttcacagtccactttagttaccagctggagttctcctgtcttgggattaatccaaaatacatttggatactggaggctggcccctccagtggagatggagtacaggaggctgctctgggggaggtctttatcagtggctcgcacctgtcccactcgggttctggcgggccttctttctgacacatcaaatacataggatggcctatcaaaaatgagaggaaactcattttctgggcttgttaggatataaacgtagacgttatttttatagtaagggggggccacatcctgcacctggattatcaccgtatatttattgccggctgctaggttacttggattttcgtagtctagatcaccaatcagcacaatcttcccagagccagctggatcctgtaaaaatctgctgccgctccccactccagatggcatggtgaagttgaatctgttgtttggtgcctcactgtcatcatcaaagcagaacttgtttaggtcaagaagcaacgtccccttggctgttctttccggcaccataatgctgaaggtgaacttttggcatgtggcaggattgtcgttgacgtcttccacaatgaaggttatctggatgcgattctcctgacccccatatggtctgtccttcactagaacttccagggaaatggtgggattttgtctcaattcacctgcatctcggtctatcctttgggccacttggattgtaccagtcaactgatttatcatgaaatatttgctaacagtggtaatgctgtagaggaggtggctgggaaaaccttcatcatcaggatcctccgctgtgatattggccacgatggttcctggactcagttcctccaggactgtgtacactcgtgtcgggctggtaaagcgagggacttcgtcgttgaggttcacgatgttcacctggagctctgtggaggctttgaggcctccactgtccctcacctccacgatgagatggaaacttctgtgtcctgcttcaaagtccaattctgttgtggagaagagggtgccattagcagacattctgaagctctttgggggagaaatcaggaaataactgaggggaatgtttcggcttgtgtcttctggatcgaaggcctcaacctggtaaatgaatccagggtttgctctttctactatgtagaggtgtagaccttctgccaagttgccttgaaactgaggtggctcgttcacatctgttacctggacagtcaggacttgcaggtctgtgacaccaacctcatccttcacataaatctgcaaatcaaatatgtttggtcctgtttcaaaatctagttgttccatcccagtggtgacaacctcaaagtaggtgcctgacagccaattcaccctaaaagcttcagtgaggggatttgagttgactatctggggaaatcctgggatcacaggtgacaatgatgctgataacttcacagaaaacttgtgcactgaagtcccaggtggagaattctctgccacattgcctgtagcaggtaagaggattaggtgtagtgcttctccccctgacatggcacccaggagagccaggagaatgattgcttcctgcatacttgatggtcacaactgtgcgtgcttccagcacattagccacagcctgaatcccgtctcacacccaaagtttatt

SEQ ID NO: 15953 - RNA, 3383 nt, Homo sapiens
  source 1..3383: mol_type = other RNA
gctgggattacaggcatgagccatcatgccctgcctgtagttcacttttaagtatattttttaaaagtaaaaaatctgaagcagctgccacccaagtgtagaatagataaattgtgatataatcatagaatgaaaccagacataaccatgaagagaactgaactactgctagacaggacaacgtggatgaatctcacatgcaggatgctgatccggacaccacaagaaaaaacaaaagaaggtgcctactgagttttcttctttccagatgaccaactcttaacttactcatctgtttttttcactgttctgcttcttttgaagaagatttgaggtgacttacaaaggtgtatggcatatttataactgaagaaatctgggtgatgttaaaacgagggcaggaaaataaggtggaaaccagatgtaaggatagtcttcactatttatgtcaggaattcctacaaactttctatggtgaacagaatagagcttcctagcagtcaatgcaaagaagaaacacaacaattccacaccccaaagttaacagtcttgcttatcagaagcacaggtagttctgaaatctgatagaaaatgttcctgtatcatttcagaacacgcaactatgtgatcaaacccctttctatttgtttaaaaatttgtcaaacatcccatgtttgaccctggatgtctgaatcccctcagcccacattttcccccctacaccatgcccacaccatccccatagaatttagggtgaggcagcatctcagtgattgacaggcccctccttagaccccgtttactttcctgggtgtggtttggggtaagccctgttcatgaaggctggatttctgttctttgggttgcccagcttgccaccctcatttctggaacccagaccagcatcctcagcccacgctttgccactcagctcatcttcttcccagttggcacttctcagtgaccccatcccttccccagcagtgactctgcgtggggcagctccctggtggctggactctttccattttggcatttgggttagtggatctttccactttctggctccagtttttgagttgaattcatatgtttccccggtcactggatctatggcttctccatcaaagatagtgttcatctggatagtttccaccacgacgtctctctctgcagtcttcgtttctcctttctttgtcagaggttccttgttcttcccagtcttgcaggggcagtgtctgtggatggctttggccaataggacgaccaggtacacgaggagacccagaagcaatatggagcccaaagtgatgacaaacggcacgtaccatgcagatggagagtaaacgtttttcctcaggacctgataggtgaccctgggctgggccaatggaataacggaaagatctggggctggaatcaaggtcggtacatgtcagcttgaaattctgaatatttgtgccaactttcagatccactgggagggccaggaaataagagtttggagtacaaattggcttttcatcattttcttcaaggatgttcacagtaacctgcagatgacaccgagttgtttttccaggaaggtgtggatttacggtgtctccatgtgccaccttgcctgctgccccttgtaaatggaacttctttaactagtgacagagcttgtgtcttcgttgttggtggcctggattctgagaatatagatgggggttgtttcacagtccactttagttaccagctggagttctcctgtcttgggattaatccaaaatacatttggatactggaggctggcccctccagtggagatggagtacaggaggctgctctgggggaggtctttatcagtggctcgcacctgtcccactcgggttctggcgggccttctttctgacacatcaaatacataggatggcctatcaaaaatgagaggaaactcattttctgggcttgttaggatataaacgtagacgttatttttatagtaagggggggccacatcctgcacctggattatcaccgtatatttattgccggctgctaggttacttggattttcgtagtctagatcaccaatcagcacaatcttcccagagccagctggatcctgtaaaaatctgctgccgctccccactccagatggcatggtgaagttgaatctgttgtttggtgcctcactgtcatcatcaaagcagaacttgtttaggtcaagaagcaacgtccccttggctgttctttccggcaccataatgctgaaggtgaacttttggcatgtggcaggattgtcgttgacgtcttccacaatgaaggttatctggatgcgattctcctgacccccatatggtctgtccttcactagaacttccagggaaatggtgggattttgtctcaattcacctgcatctcggtctatcctttgggccacttggattgtaccagtcaactgatttatcatgaaatatttgctaacagtggtaatgctgtagaggaggtggctgggaaaaccttcatcatcaggatcctccgctgtgatattggccacgatggttcctggactcagttcctccaggactgtgtacactcgtgtcgggctggtaaagcgagggacttcgtcgttgaggttcacgatgttcacctggagctctgtggaggctttgaggcctccactgtccctcacctccacgatgagatggaaacttctgtgtcctgcttcaaagtccaattctgttgtggagaagagggtgccattagcagacattctgaagctctttgggggagaaatcaggaaataactgaggggaatgtttcggcttgtgtcttctggatcgaaggcctcaacctggtaaatgaatccagggtttgctctttctactatgtagaggtgtagaccttctgccaagttgccttgaaactgaggtggctcgttcacatctgttacctggacagtcaggacttgcaggtctgtgacaccaacctcatccttcacataaatctgcaaatcaaatatgtttggtcctgtttcaaaatctagttgttccatcccagtggtgacaacctcaaagtaggtgcctgacagccaattcaccctaaaagcttcagtgaggggatttgagttgactatctggggaaatcctgggatcacaggtgacaatgatgctgataacttcacagaaaacttgtgcactgaagtcccaggtggagaattctctgccacattgcctgtagcaggtaagaggattaggtgtagtgcttctccccctgacatggcacccaggagagccaggagaatgattgcttcctgcatacttgatggtcacaactgtgcgtgcttccagcacattagccacagcctgaatcccgtctcacacccaaagtttatt

SEQ ID NO: 15954 - RNA, 1946 nt, Homo sapiens
  source 1..1946: mol_type = other RNA
gctgggattacaggcatgagccatcatgcctggcctatagccttttgatattcctgcactggtaagatacagaattagggaagatggagggtgaactatctatatatctggagatagcttggaaactccaatagcttctgctactttgttatgttttttatatgtttttgattgtaatcaaatcaagtgttttttattacagtaggtgaagagtaaatgtcagctcctgctgtccctgtctaatctcattggtgtggtttgcacacagtacatgttcagtccatgtcagttgctgctccttgtgtctaatctccttgttgggattgtggacacagtaggtgtcgagcggatatcagtaaatgtcagctgatttggttcatgtctagtctcattgtatgttacgactttgcagcattcagcttcttgagggcacgggggaggcatgaacacagatgtcatttcccatgcagcctatgaacttggttgatggtgggtgatgctctgagtactggactggggttttcaattgtgtgacaccagtgggtcacttcagcctgatacagtccacctcttctgtggtgggcaccccgttggttctgaggtcaaggtcagcactggacttgctcccccgctgggagggacgccagtgcagcagcatcatcttcttgaagtacttcatggtgttgttcttgaccgtcacgaagcacacggtgttgatcatgctgttgctcatggcgatgcactcgaccacgtagaaggcagtgaggtagtgcttttccttcacgaacacagtggggaagaagtcacgaacgatggtgaaaccgtagaagggtgcccagcacagcacataggccgtgagaatgcacatgagcaccaggaccgtcttcctgcggcagcgcagccgcttgcgaatctgctccgtctggaacccagggactgccttgaaccagagctcccgggagatcctggcatagcacagggtcatggtgaccacagggcccacgaactcgacaccaaagatgaagaggaagtaggacttgtagtagagctgctgatccacaggccagatctggccacagaagatcttctcctggctcttgacaataaagaggaccgtttctgttgcaaagtaagccgatgggatggcaatgagaatggacaccatccagaccaaggcgatcaggaaggaggccgtttgataattcatccgtggtttcaaggggtgaacgatggcgagatatctgtcaatggcaatggccagcaaggcattggtggagacgtagagggagacggtgcgcaggtagttgacggaggcacagagcacgtggccatgctcccaggagagctgccgtaccacgtagtagtccatctcgaaggggcagcagatgatggccaccaggaagtcggagatggccaggttggcaatgagcagattggtgaggttgcgcaacttcttatagcgggtgagggcagcgataaagacaaagttaccgatgccgcagaccagcatgatgcctgccagtgcaatgccaatgacgatcttggctgcgaagaaggtccgggtcttggtcatgtcctcatcctcatccatagggaggtcataatcaccataactgaagttaaaggagagggaggaggcatggtcttggggtggattaaagttgggtgtgaaactggtgtttccattctgggctgccatggtgatgtctgtctcggcgcctcctttctgtgcgctctgctgctccggaagccggatcgagagtcacagtgtggttgggcgcaggcgggccgctcggttttcacctcgaggacccggacttgcacttgcagagccgctgcgtgggggatgtccctcttttttcctcgccccggcgggctcctccggcgtgtcagggtctctgggttccagctggagttggcgctccggccccacagctctttccagc

SEQ ID NO: 15955 - RNA, 2168 nt, Homo sapiens
  source 1..2168: mol_type = other RNA
gctgggattacaggcatgagccatcatgcctggcctatagccttttgatattcctgcactggtaagatacagaattagggaagatggagggtgaactatctatatatctggagatagcttggaaactccaatagcttctgctactttgttatgttttttatatgtttttgattgtaatcaaatcaagtgttttttattacagtaggtgaagagtaaatgtcagctcctgctgtccctgtctaatctcattggtgtggtttgcacacagtacatgttcagtccatgtcagttgctgctccttgtgtctaatctccttgttgggattgtggacacagtaggtgtcgagcggatatcagtaaatgtcagctgatttggttcatgtctagtctcattgtatgttacgactttgcagcattcagcttcttgagggcacgggggaggcatgaacacagatgtcatttcccatgcagcctatgaacttggttgatggtgggtgatgctctgagtactggactggggttttcaattgtgtgacaccagtgggtcacttcagcctgatacagtccacctcttctgtggtgggcaccccgttggttctgaggtcaaggtcagcactggacttgctcccccgctgggagggacgccagtgcagcagcatcatcttcttgaagtacttcatggtgttgttcttgaccgtcacgaagcacacggtgttgatcatgctgttgctcatggcgatgcactcgaccacgtagaaggcagtgaggtagtgcttttccttcacgaacacagtggggaagaagtcacgaacgatggtgaaaccgtagaagggtgcccagcacagcacataggccgtgagaatgcacatgagcaccaggaccgtcttcctgcggcagcgcagccgcttgcgaatctgctccgtctggaacccagggactgccttgaaccagagctcccgggagatcctggcatagcacagggtcatggtgaccacagggcccacgaactcgacaccaaagatgaagaggaagtaggacttgtagtagagctgctgatccacaggccagatctggccacagaagatcttctcctggctcttgacaataaagaggaccgtttctgttgcaaagtaagccgatgggatggcaatgagaatggacaccatccagaccaaggcgatcaggaaggaggccgtttgataattcatccgtggtttcaaggggtgaacgatggcgagatatctgtcaatggcaatggccagcaaggcattggtggagacgtagagggagacggtgcgcaggtagttgacggaggcacagagcacgtggccatgctcccaggagagctgccgtaccacgtagtagtccatctcgaaggggcagcagatgatggccaccaggaagtcggagatggccaggttggcaatgagcagattggtgaggttgcgcaacttcttatagcgggtgagggcagcgataaagacaaagttaccgatgccgcagaccagcatgatgcctgccagtgcaatgccaatgacgatcttggctgcgaagaaggtccgggtcttggtcatgtcctcatcctcatccatagggaggtcataatcaccataactgaagttaaaggagagggaggaggcatggtcttggggtggattaaagttgggtgtgaaactggtgtttccattctgggctgccatggtgatgtctgtctcggcgcctcctttctgtgcgctctgctgctccggaagccggatcgagagtcacagtgtggttgggcgcaggcgggccgctcggttttcacctcgaggacccggacttgcacttgcagagccgctgcgtgggggatgtccctcttttttcctcgccccggcgggctcctccggcgtgtcagggtctctgggttccagctggagttggcgctccggccccacagctctttccagcgtctcggacctgtgcgccccgccccgcgctggactccgccccggggtccccgcctgcctcctagtccaggccaagggtggatgcccagctcccccaccccaccgcgtgctctcgggctggtgcgtccagggcgcgggcaccgtagctccggccgcgctgacgcgagtccccggcagcgggggcagcctctcgcacggatttcagcgccttcgcatcccgtct

SEQ ID NO: 15956 - RNA, 5062 nt, Homo sapiens
  source 1..5062: mol_type = other RNA
gctgggattacaggcatgagccatcatgcttcatgctattgtactttttaactatacaatttttttggttcttttcagttccataatttctgtttggttccttttataatttctatctattaataatctttatttttttaaataatttcaaattttattttagattcagagggtacatgtgcaggtttgttacctaggtataatttgtgttgctgaggtttggggtatgactgatcccctcacccagatactgagcattgtaccaatagttttttcaacccttgcccttttccctccctccctgtctagtagtccccagtgtctattgttgccatctttatggtccatgagtacccagagtttagctcccatttacaaatttgaacatgcagtatttggtttttctgttcctttattaattcgcttagaacaatggcctccagttgcatccatgttgctgcaaaggacatgatttcattctttttatggcttcatagtatcccatggtgcatatgtaccacattttctttatccaatccattgttgatgggcacctgagttgattccatgtctttgctattgtgaatagtgctgtgatgaacatactagtgcatgtgtctttttggtagaatgagttcttttcttttggatgtgtacccagtaatgggatagctgggtcgaatggcagttctgttttcagctctttgagaaatctccaaactgctttccacagtggttgagctaatttacatccccaccaacagtgtataagcatttccttttctctgcacccttgccagcatatgttgttccttgactttttaataataactgttctgatggtatctcattgcagttttgatttgcacttctctgatgattagtgatgttgagcttttttcatgtttgttgaccatttgattattcttttgcatattccctatttgtttttgagaccttgttctcctggttgtttctttccgatctttttctatgtttcttttcactttttgttcatgtttaagacaggtcatttaaagtatttctcttataattcctgtatctgcacttcctcggctcagggacagtttctgttcatttactttttcctttgatttggccattttttcatgtttcttttttttttttttgcatgcctcataattttttgttgaagattggacattttgagcattataatgtggtaactctggaaaccagagtctctctcctcccccaaaatctcttgttgtttcttagacaacactatagagtaggttgtaattatgaaacttggtaaattacggtgtccccaatccccttggtaataaattgtggagtcaggattcaaagccataccttttccactgtattctctactctatcctttctattctcattttattcagtaccctaaaaatctggatcttccccattgctttattcccatttcagtgaatctcagatctgtatctccagccctcgcctctcttgagtggcagataaatgtatttctaactagttacaaaaatatatttctaactagttacaaacactatcacgaatttcaaactcaggaagtcttaaagtaaatttattatctcactctcctgtttccacgaactttcccgaaattttcttctttcccgcccttgcgaatcccttgcatttctcagttaaaggacagcaccatccacccacctctcccaaagccgagctttggatttatcctcattggctaaatccctcctgaaacatgaaactgaaacaaagccctgaaccccctcaggctgaaaagacaaaccccgcctgaggccgggtcccgctccccacctggagggacccaattctgggcgccttctggcgacggtccctgctagggacgctgcgctctccgagtgcgagttttcgccaaactgataaagcacgcagaaccgcaatccccaaactaacactgaacccggacccgcgatccccaaactgacaagggacccggaacagcgacccccaaaccgacacgggactcgggaaccgctatctccaaagggcagctttctttgagggaggctgttagacgtgactccttgtttctaaaaatggacaaataccagcctgggcaacatgacaaaaacccatttctagtaaaaatagaaaaaaattagccaggcatggtggtgggcgcctgtaatcccagctacgctggaggctgaggcaggagaatcacttgaaccgggaggcggaggttgcaaccagctgagatcacaccactgtactccagcctgggtgtcagagtgagactccatctccctcccaaaaacacccaaatgcagaatatatatgtgtatatacacatatacatattccatttaaacatagttgtatatttttattaccaattgttcggtttttctccagaatgtcttaacagaaacccacataatgagtctttttgaatgcatagaattatatacaaaaacccatgtttcactatcacataatgttaatttttaatttagaaataaatgcttctatgttcttgagtcacacaatctgtaactaaaatctgtcatgtttttattaagatgtatattataagcctgtacaaagggattttgggtgttgtaatatcagccacaaaagctagaaatcattcttaaaccaacacacatgttgcaagctatgatattcaatttttacaatgtgttcaatttacaacatgattacaatgtttcttaaggtaatgcctaatttttccagtttgtatgtataacaattctaaattcactgtcatattgacttaagagagggtccttaaaaactttgtttcctacaggatggtgatgggaatctttgcaaattgtatcttctgtttgaaagtgaagtacttacctcggcagcagaagaaaaagctacaaactgacattaaggaaaatggcggaaagttttccttttcattaaatcctcaggtatttccaaatgtcataaactacagtgtgataaaacatcgcgcattcagggaacaacagggtcatggttagaagaggaaacagagattagcagcaggagagagtgagctactggaagctcatcaggagagactgtgacttggccggttgggaggctgggcccccagaggcagaggaggaccagccctgttctctccctgttccctgaaccgcaggacaattccacatgtccagtgaggcaggatattactagagcacagccaaatatgaaaatagaatttcagaccagtcaaatctattcttgaaggaaaaaagtcatagtgcacaggatttgcaaaaagcgcactgtcgtcactcaccagtgtgtcaacgctggggtgatatactggtaagccaggttcctgggggcaaaaagaaagatatgtagtgcagactcatcttcgcagtgtagcttgtgctgtttgttttgttcatttaaagactgcaggaagctacattccatcttttgaattgaacttgtaggcctggcagttcagataacaggatttcacaactggatgaaatcttggaaacagttaagtctaacctcttcttctttttttttttttagatggagtctcactctgttgcccaggctggagtgcagtggtgcgatctcagctcactgcaacttccgcctcctgagttcaagcaattctcctgcctcagcctcctgagtggctgggattataggtgcctgccaccacgcctggctaatttttgtacttttagtagagacaggatttttgccatgttggccaggctggtcttaaactcctgacctcatgtcatccgcctgtctcggcctcccaaagggccgggaatacaggcatgaaccaccgtgcctggccccctcctctttttttaaaccacctcgttgtaagaagtaaaaatagaaatccaaaggctctaggttccaggctggcctgcccctgtcctctcctgttccctctgttgatgaattgatgggctgactcagcctgcccctccctggacctcagccctgggacttggccatagtgagcctcatctgtgaagcgtgttcaactccagctgaataccagaaatgcaatgtccctgtttacttccaattcaggtagaattgtatatacttcccttatacagcttcccacactgagctgtctcaccatctctgtggacagatgagtaattcgtgcccgctctcccttctcagtttgtcttctgtgtggagaactgccaacatggtctctcctttttagaaactcacatactgtaagtgcaaccttttggaagtcagtgtacataaacatgtgaaatgtgcatcccagctactgtagataatgaggcagctctacatgtaatcacgaggaaaaatcgccaagataaattcagtggacaaaccagcacggaagaggctgaggagcacgctgccatatgtctacacatagtgtagctctagcagaattcgtgaggagcaagtgacagcaggtgcctctgcagaaaggaactgtaatcccagttactcgggaggctgaggcaggagaattgctcgaacgcagaaggcagaggttgaagtgagcaaagattgtgccactacactccagcctgggtgacagagtgagaatccaccttctgacatccagaagcttccctgtgccagatggagccaccaatgtggggaggagagcacaaagagcagagaatccacagaaaccataccaaaaagtatctccacggcaaattctggtggataaattttccaagctttttgtttatgtggattatccaattcatttcttggtagataaagcctttccactggagatccacgcaacccgggcagaggaagagattgtttctcccaaaccttgacgatcatttgaggaaagacttggagactttgtgggggaaagacacagggaaacgctgccggcattgtcccaaacctggactgggagcaggacaacactgggggaatcttccctatctggctccacccatcttgtgcccccaatccccctacccctagggctgagggagctcagattaatgtgtactcaggaaatcagcccatt

SEQ ID NO: 15957 - RNA, 7447 nt, Homo sapiens
  source 1..7447: mol_type = other RNA
gctgggattacaggcatgagccatcatgtccggcctcaagttatattttaatagcatacaggatacatactcgtactcagaatgtgagttcaaggatcagtggcacaaataggggaaatgacctcaagttccaaatgttaatgtagttctattagagtgtctgagtggggagaaatcatttcttgaattttgcagggcaagcataagtgctttgactcatttttgtacgcctcacagcgtgcttgtaagccatgtctccagggccatacactcattgtaagtgcccctaataataataaagcaaaggatctgctgcaactcaaaggaaataggaagtgctttaagttccacattccaaagtcagggctagagaggcaggctggatttcctgctgatgtggattgcctgctgttggtttgggccattctaggtataaggtaatgttttagattactgctgggttcttctgggcctggcaacataaagaacaaatctaatcaatgcatcagctgctatggctcattcaccttcctgaagtgttgtgtggccacagcctgcaagaatatgacctggaaatccccaggtagggccctcgggtgtgctcagatccctcatgcccacccatccacccctctgcattctaacatttcagtggttatgttcaggcaaagtgtcttctgctcatgcttgggaggaagagttcccttaacctccctgtggctcattgtccctgaggataccagggctctctcagcctggctgcatgatgacagagggacaccattatcagagaaaccagggctgatgagcagctctaggtcagagaggccgaatgctacctggacatgaagagagaggtcccagcagaccccctggggacaggttcaaattaggttccagcttccccttcctggtgtcaggagttactcatcttgatttacttatcttgcaaaggagccaaggtatcctgccgtacctgcctattgccttctgtctcttccacaactcccatgtctcttttcggtttctgctccacttctcatgggctacttggagtaggaagtaggtctcaataataaaaaactaaataaaacaaaaacatcatctgatttgcctccagctctgccacagactatttggccctagaacaatcccttccctttcctgatactcctctgtaaaatagcctggatcagtagctttcatattacattctgtgaagctgccaggagccggaggggttccccagatacccggagaggctgcagtggaaagacaggctaagctgactccacccccaacacccagcgcccaccagagtagctgccttttacctgttttatatattgtttttccacacagagcttctttgaagaaagagtcctgaggctacaaaatttgaaaactgctggaataaacgatcgccaaggccccttccagtctgagacgcttggtcttctgaagcccagctcaagtttttcctcctccagaaagcctttcttgttacccagtcctgggtacttgagctccaacaataatgatgatggcaggcatatggtgccgtccgtgagccatccgatgcctgcatgtgtgcataagctgtctccccagctagaaggtgagctctttgagggtggtgttcaatttttcttccacacctctgtccccttgtaataccatatgcaaagtaggtgttcaataaacatgttgatgccacctggtgtcatgagctctcacatgggataaaacttccctaccaggaagtttgggaaggaggaaccagcctttggtctgcttaacgctccacagagagacttgtccttaaaaagctggggaccctaacctgggaagcagcttcagactcatacacttcccaaagggcaggtctgagttcctgccttgattggatttggcttcacctcttctgcccctcagtacctcttctggtggggcctcttatacactgtggctgtagaagaggcacggtcctgaagcctgggaatcaggtcagctaggacgccccagggccagcagacatctcagccagattccagagggaggcacgggggagatggagaggaactcctgggtttttttggaatacagctctctcaggaagtggaggcccaaagagggtggctggattcagtcagagacaccagagaaagcagattggaggagggtgctagcggtgaaagaaggcaggtagccaaagggaaactggaggttgtagtggtggaatgaaaccgctctgccatttagtggctaagtgaccctgaggtcagttcatcttacttagtctcaatgtctttacctataaattgggtgtcaaaagaacctgaccaatgtcaggctaccctgtagtgaagtagtgagatagattccaaggagactaaaatgtgcagagatggaaaggattattactgtttattaacacaggaaagcacaggagcctgcttccaaagagggactgtcccgtaattgagagatgctccaaggctgaccatcctccttctcctgctgcacacccagcagccatctatggctggatttggagaatttctggtcaaaccggtgagtatgaggagagcagggcagttggggagagaggtcccagcccaattctgcccagagaagctcccaaaagagagggaagtgtcctgatgaagagcccatgaaaggggtgagacccaggaggctgtggagattgctgcgggctcctctggtcagtaaggaaccctgacaagatccctaggatgggggtcccttagtctcactgaagttcttgtaacttgggatgggggccaggtcagcctcctctgatacccgaagctacacatctggccttccccacttctagaggaggggtcttagatggtgctgtgggagcagacaagccctcagcaggtcgcaagcaggtcccctccaaaacccctcctgctggaatcctccagatgtgaggagtaggagcagacagatcaaggctgggacatctggcagggtttaacatccacagctggagggtgagacctctccctgtggatctggagaaataccttcgggctccagcctattgctgcccttgccttgtcatccatgacagggttccgcgccctgtccagcctccccgggtccccctcagctgctatagcctgacgtgtgagtgctgggcctgcgcagccaaacatctggcaggtctggctggctattgggcagcaccacagggctgccatcccctggcccccctcggcccttccaggacaagctgctgtgatgggaagcgggcaatgatgggtcatacactgtctccctcagcgccagccacagggtgtcccgcttcccattgagctggcctcgctcaaggactggctgcccagtgtcatccaggtcatctggggacacacccacggaatctggtacacgggcactgggctcagaggtgcttaggcaggtctcatcagagacgctgagcccctccagggtgctggctgaggaacagaagccatcaggaggatctgcagccttggccttaggagagtgggctggggcttctggtgaggctggcaggggctcagcctcctccccttgggagtcctgcctggcccgggttttggggctggggccagcctgcttatagggggaggaggtctgcagggcagggcactggctgaagactgcctggtggtccagcagcagctcccttggggaggcaggggctggtgggggccgggaacagcacggaccatcatggagctgcagatcctcagagagtactgagggccggtgggacagcttgctggtggctgtgctggtgtcaaagctggggctccgacgccgtgccaggggctgtagctcatattgctctgagcaggacccgggcatccctcccactgaccctggtcgtgggcggcctgccttctccccaccagggtccccagtaccagcatcccatggcaggtgggcacagggccagaggatctgcccacagttcttctctggcccgaagaaacagcagagagattggaagaagaagctggcaaagccacaactgacgcatttgaccatcatgaggatgatgcccagcttgcgatagagcagcactgtggcaggcagcatgagcacgcctgccgcaaacagggctgcagcccccacggctgtggcgcagctggtctggcgcagagagaaggccacacggctcaggcggtcagggtgtgggcacaggtgataggagatgcagtagttgacagtgaagtctactgagaggcccactgaggcagagagaaacagggcctcggcagtgttgagctgccactcgaggagaaccaggagtcctacagtgagcagcacggtgcctgccacagctgccacggagaataggctgaggggaacattccaggtgcccaggagcagtgtggcaaaggccagcgccaaagccaggcccagcaccacagcaggctcagtgctcaggctgtgctgcaggctatacagctctagacggctagtgaaccaaccacggcggaggcctggaggtgccatgcccagctccgctgccagccagtggctgacctcattgtagaagagctgggtctggttgtagtccggactgttccggaagttggtctggaattgtaggaccagggcggccaggctgccatgggcatcaaagcggagtcccaggtcctgggtgccatcggggccttgctccagagccatcattttcaggcagtgcaggaaaaactggggggcccaggggaagtccgagtggccgcagcagaggtcaggccccaggcgggcgcagctggggctctccatccagcgctggagggtctccacgaaacacagcgtgggccagccttcctgcagggtgtcgaagaagctctgattccgggcccggtgacagagtgccagcagccagcgctgggcctcagggccgctggccgagaaggcagggtccctcaccaggctgctgttgctacgagggtccagagggtcgccagtgtccacaggcaggacgccccacaccaaaaccacgggcatgtggccgccctcgccctgcggcagctgctcgaacaggaacagctggcgatactccgcgtcgaagcgctcgaaggggtggctgggccggaagacctggccgccgggcggcggcagcgtgggcagccgcaggcgggggctgactccggcgatgtaggcgccccctgccgccagtgctgcgaaccagcagatccagatgtagcggaacttgatgacgccgcagggcagcaggcgctggaagagcagacgcgaggtgccagccgccgccctccgcaggccgcggagccgccggtgcagcgccagcagtagccgccggggcgcgctgccctcccaccggccccgcgcccggcgcgcacagccgcgcgccaggtagcgctcgtggagcacggcggaggcgggcagccagaccagcgtgagcgccaggtgcaccagcacagccgtgcccatgaagagggcgaggcagcgaacggccggcaggcggctcaggtagctggcatagaaggccgcgctcgtggtgaggccggagaccagcagcaggtagccgaagtggtgcatggtgcggcccacgcgctgcgccagcccccccgacggcagctggctcttgctaaggcgccacaggtcgaagaagatgagcgtgtggttggcgcagacgctgctcagcaggaggagggctgccagattgacgaaggggaagtaggccatgcggaaggccacctggtaaaggaagaaggccaccagcagtgagcccagcacccccagcagcaccatgagcgtgaggaagagtgagcgcaggtacagggccatgccgaagaagatggcaaccagagccagcaaggggtacaccgtgtcctggaccaggaagtgcctcagcagctcctgcttgaggcccaggtccatgccagtgacagaggtgtagttgtcagcaagcccccagggggtggccagccggtccaggtagatgtccatgagggaagcaccctttggggtgggcaggaagagcaggctgtacttgagggaaggcacctggtagtcagtggtctggggactcagaaagtccctgtcaagcagaaagtgcaggagttggtagatggcactactctgggagcacttggtgggaacctgggcacagcgtggggacttgttctgcccaggtcccagacaagagggcaccaaggcgccactgtggtagtagagggcacaggtccgaagcagggccagtgtgcgggctgcgtcagcttgggtagtgtccaggcaggaggagcggttggagagcacagccagatagttgcccagggaccagctggggcagcactggttggctgctgtccgctggcacagagccccgaagctggtatgggagcggatctggtcctgttccatgcgacacatggaatggatggcatgcaggttccataggctgcccgaggaggtggacatgaacaccagctttgcatagctcttctcaggggggccacagaagaagttctcttgccttctgtcctccaggggctccaccattctccgaggccggacagcgctctcctgggcactgcctctgggtgcaggcctcagagtgttgtgggagctcgagctgttcagctcaaggtctggggaaaggaaaagcagcttcctggggcctgtgagggcttgtagtgctctccagaccactaacttgctcccaatgtctgtgtcccgtggctcaaagcccagcaaaggcttggagaagtcgggcagccgggcccccaacagtccagccagggtgcagaggaagatgacagccagacacagcatcagcacggccactggccactcagcaatcagctgggaatagctctttggcatctggaaggctcgttcctgcctgacgctgaccacatggtgctgcacagcgggtggcttccaggtcccatcgcgctgtgagggggctggagaagggctgaggctggagccgtgggagcagagagctgcccgatccccaagtcctggcagggaactgcccccctggtattcctgcagtgcccggggataggtgaagtgggcaggggccaaggggctggatggacccacaggctggagggtggaagttgttggtgggggtcctgaagagctggaagggtcctccagggggcagctgtggagggagcagcttctctctgggcttgcctcagggggcacagccttggtctgggtgctgtccggggagccgccgtctggggccaagggctccccctcgggccgttgctccccttccggacccgggccgggagccggaccgctgccgccgctgctgctgctgctgtcaccgtccatgcccgtgggcggcaccgctgtccgggcgctggtgctgaagccgcggcggcggcggcggcggcggcggtggcggcggcagcggcggcggggtgctcgtgcgcat

SEQ ID NO: 15958 - RNA, 5167 nt, Homo sapiens
  source 1..5167: mol_type = other RNA
gctgggattacaggcatgagccatcctgccaggccataacggagacttgaattcactatcccaaggccctgagagctccaaggttacaattctgccctgaggctccagtacaagtcttaggttttctcaagtgtgagtctgttggaagtcttaggaggtttgatatttgggaacatcatgacccaacgtggaccacataattatatctaccaggcctggacatctgggttacacacttctattcttcatatacctgagttcgtgtacattcataggtatttttaaagaagaacccttctccccacagtctccaaaatataatattgttcaaaatactggtctaggaaatgaaacactagggtaacaatctttaaagacttacaaaagcaactcagtattttgacacagatgacacagaagagtcacatgaactcacagaggatcacatgaggcctggtgggacgaggtttctctagtactttccactgggcttagaatgcaaaaggctctggctggacttgctggaggtctctttcctcagcatctctctttcttggtccatctttagggaggcttttctggttccaacctgggaatttgagttctgcatcctgttcttcaccatctctacaaatactcgtctctgcctgtctttctctttgaaggcacagttgcaaggtgtcgattcttttgcgtttctcagttcgtgctcctctacactttccttctgctgccggatggccctgttgatcctcttctcctggcacagctggtgctccatgcgctccagggcctccttcagcagggccttctcttcggcctctttgtagatatcatcctccagctttgccacctgcgactggtacatctcaatggacactttgctccgcctgagctgttcaacgtccttttcatatcctctcaacagctcctctttcctccccagctggttcttgagttgggtgatcttatcaaacaccaggtcgaggtccctttgtcgaagctggttgaccttctccctctcctggcgggagaggtatttcatggacacgtggcctgacatattcttgatgttcatgagacttccgagggttttgctcatatccaggtacagcttttcactgagctctaaagcctcagccacatccatcttccctgacttctccatggctgagccgaaccttgcgttgcaaaggccattctgaggcgctaggatctctattcttgagagagttggcaaatccggttttgcatccagtagtattttctggacattgttttccattctgaggttctttaaatctagaaatgattcattctggtggtctttatgatctggtgagcgcgccttctcgagttctttaattcgcgctcgaagttcagataaggcctttttctgacgctgaatgacctcctcgtgccgggaccctttgcacctgacccctagatcgctgaaggattgctgctcttggctgctggagaaggcctcagtgtggacgggttctatctgcacagaggtgtcacacgtctgggtcttcttccggggcttctgttccttctctgtgttcagctggagtctgtgtttctcttgggaagccctgagtgcctcctcaagggccttcagctcccgatctttcttttctaccaggctgctcatctgggccatcttctccttgagcacactcagctccttgctctgctgctggaccagcaccacgttctgctccagttccatcttctgcttctcgtttagctcccctctcaaatccgacattctgctgtgggcttcggtaaggtctttccttaacttcatgatgacttcctgctgagacagaatttccttctgagcagccaataagtcatctatcagatgttcgtacgccatgtctttggcactgctctctgtcatgggagccaccagagggtcttgcggcctttcctcctttggggctgggtcattgtccttcaatgttgcaatctcgccttctatttttttatggtgctgagtgactttctggagtttctcttcgaggctcacaattgtctgggcgtgctgtttgatttgctccttatattccatgatctcttcttcaaacccgtgtctctgtgattcctgctcatcctggagggcctttaccatcttctgctgcaggattagccgctcttccaccatgatcatttttgtcttggtagtttccagttcggctaatgtttcatttaatttcaaggcgaggctctctgcttttagactttcagttgcctttgttttctgagtctcttcaaccatggccagtgcgtcacttaatttattatttaaaacgtcctctttttgctcttttaattctaattcctctttctgcttggttaagcgattctccaggtcttgcacctttttcttttccttctccatggcctcctttgctttgcgtttctcgtacgcaatgttgctctctgagatctccttctgttgggttaaatggttctccagatcctgaacttttctcttttccgactccaaggcttcctttgcttttcttttttcatgggctatgctgctctccaaaacctccttctggcgggccaagcgttcctccagctcttggactcttgtctgctcttcctctaatgcttccttcactctgttcttctcctgggtaatgcttttcgccaaagccttcttctgctgggccaggaggctctccagttcttgcattctcttccgttcttcctctaaagtctctttcgctctgtttctctcttgagtaatgtactcctccaaagccgccttctcttccgtcagttgcctgattttggctttgagcttctcctcttgctctagcctctcctcgttcagcttctccttctctgccagatgctcccgcagcttttcctgcagtaaagactgctgagtttcctgagaactgttgaacttgatctgaagttcctgggcctggctcataagttttttataatgttccagaagatatatcagatacaaagagaaccctttgttggggctggagggcaggatcccgaggtcccggaggagctgctccacctcctccagccaggacagcgcgtgcctcaggacgtccagcaccaccttctggagccccgagacaggtgggctcacctggaggtgctgaagaaggtcgacctccttcttcaggtcatggctgcaacaggatattttcatgcaagcctggcagctgtccagcgacgtcctcagcttctcgatgttctcggtggtctcctcctgcttggagttgctcagctgggtctctttctggagggtccactttttctgctgaaaattgatgttgtcctcagtgacctgggtaattttctctattaactgttggtcggtgacgggcttgtcccggaacggcttcgcccgtccataggtggccttgatgacttgacttctgaagtgctccagctgacctactgccctctccaaattgattttaatgacgctctctctgttccccatttcttgcagctgaagcaatttccttctggaatcctcctgaagcttctcttcaaccttgcttttttctctcagagtcctagagatcacgctttgttcagtacaactcttcctcagctctgccctaagcttcttcatttctttctccatgtcttggatttgggttttgcagagttttaactctttctcctgggcttccctgagctccctgtgagcatcttcctgttttaactcttcctttagcaccgagcatctagagccaagggcttccagctggtggtccttgtccttgttctgactttttaggtgactgacctcttcctttagttgttgaacttgctcatcctttgctaatatgtctttttgcaaagatgacaccatccctgatgtgatagcgttgtctctctttaagttctcgccctcattcttcagggatgtgatttctgagttccgctctgacagggtctggcacagcaccttgctgtagcctttctgtagggcactgatctggcttttcaagctctggatctctttctgtttggcatcgatgtcttcatccagaacctgacacttctgcgagatctccttctcattctgcctggaggtggtggtctctgacaccttctgactcagctcagccacttcattctgcaggtttgctattatgacgtctttgtatttggattcaatttcataatctgagagacggctgacctcttttcccagcagcagaattatttcatccttgtcctgctgggccaagtcctcctccacataaatctccgcagggggaactgccccaggaatcccctcggccactgatttttctgacagtttcatggcattggtccacacttgcttgatgacgggtggcttgcgggcgtcgtccaccacgaacgagaacatctccttgttggcgctcacaggccgcctgtgggaggccggcaggaccacggtgggtctgggaaaggcctgggaccagctcctttgcatcggtgctggctggacaccttggtggaaggggatatgtgatggtgggggggcctggtttggctgctgtgtggcacgaggtggctgtggccctggccatggtgctgggcccctcatccatgggaaagagaccggaggtggattttcaatgaccagttcataggtcagccctgcagacccaaatctcaggatgtctccagggatgagcttcacagccacgttttgaatgtggcactcgttgacaaacgtgccgttgcgggaattgaagtcctggagaacaaagctgcactccgcctcgttatattcaatgagtgcatggtggttgtcgatgtcaggagactgtaaaacaaggtctgaattttcatgccttccaattgtggtacttttatttaggacaaaaaagccttctgcgctctttagataggccttcatcctctctgttttcccgtaaatgaaaagtctgcagggctcaagtgatgtcatcagacctcagtctctctctggctcctcagcaatacttttgaccacgtggatccaacctcagacagaatctctgtataatggtcccagaaagactgctgcagctccagtccttacatcttctcagctttgaatcccaaggggatgagagagaattttttcctaagattctcccaaaggcctcatggcttctcattttctctgatt

SEQ ID NO: 15959 - RNA, 4896 nt, Homo sapiens
  source 1..4896: mol_type = other RNA
gctgggattacaggcatgagccatcctgccaggccataacggagacttgaattcactatcccaaggccctgagagctccaaggttacaattctgccctgaggctccagtacaagtcttaggttttctcaagtgtgagtctgttggaagtcttaggaggtttgatatttgggaacatcatgacccaacgtggaccacataattatatctaccaggcctggacatctgggttacacacttctattcttcatatacctgagttcgtgtacattcataggtatttttaaagaagaacccttctccccacagtctccaaaatataatattgttcaaaatactggtctaggaaatgaaacactagggtaacaatctttaaagacttacaaaagcaactcagtattttgacacagatgacacagaagagtcacatgaactcacagaggatcacatgaggcctggtgggacgaggtttctctagtactttccactgggcttagaatgcaaaaggctctggctggacttgctggaggtctctttcctcagcatctctctttcttggtccatctttagggaggcttttctggttccaaccttctgctgccggatggccctgttgatcctcttctcctggcacagctggtgctccatgcgctccagggcctccttcagcagggccttctcttcggcctctttgtagatatcatcctccagctttgccacctgcgactggtacatctcaatggacactttgctccgcctgagctgttcaacgtccttttcatatcctctcaacagctcctctttcctccccagctggttcttgagttgggtgatcttatcaaacaccaggtcgaggtccctttgtcgaagctggttgaccttctccctctcctggcgggagaggtatttcatggacacgtggcctgacatattcttgatgttcatgagacttccgagggttttgctcatatccaggtacagcttttcactgagctctaaagcctcagccacatccatcttccctgacttctccatggctgagccgaaccttgcgttgcaaaggccattctgaggcgctaggatctctattcttgagagagttggcaaatccggttttgcatccagtagtattttctggacattgttttccattctgaggttctttaaatctagaaatgattcattctggtggtctttatgatctggtgagcgcgccttctcgagttctttaattcgcgctcgaagttcagataaggcctttttctgacgctgaatgacctcctcgtgccgggaccctttgcacctgacccctagatcgctgaaggattgctgctcttggctgctggagaaggcctcagtgtggacgggttctatctgcacagaggtgtcacacgtctgggtcttcttccggggcttctgttccttctctgtgttcagctggagtctgtgtttctcttgggaagccctgagtgcctcctcaagggccttcagctcccgatctttcttttctaccaggctgctcatctgggccatcttctccttgagcacactcagctccttgctctgctgctggaccagcaccacgttctgctccagttccatcttctgcttctcgtttagctcccctctcaaatccgacattctgctgtgggcttcggtaaggtctttccttaacttcatgatgacttcctgctgagacagaatttccttctgagcagccaataagtcatctatcagatgttcgtacgccatgtctttggcactgctctctgtcatgggagccaccagagggtcttgcggcctttcctcctttggggctgggtcattgtccttcaatgttgcaatctcgccttctatttttttatggtgctgagtgactttctggagtttctcttcgaggctcacaattgtctgggcgtgctgtttgatttgctccttatattccatgatctcttcttcaaacccgtgtctctgtgattcctgctcatcctggagggcctttaccatcttctgctgcaggattagccgctcttccaccatgatcatttttgtcttggtagtttccagttcggctaatgtttcatttaatttcaaggcgaggctctctgcttttagactttcagttgcctttgttttctgagtctcttcaaccatggccagtgcgtcacttaatttattatttaaaacgtcctctttttgctcttttaattctaattcctctttctgcttggttaagcgattctccaggtcttgcacctttttcttttccttctccatggcctcctttgctttgcgtttctcgtacgcaatgttgctctctgagatctccttctgttgggttaaatggttctccagatcctgaacttttctcttttccgactccaaggcttcctttgcttttcttttttcatgggctatgctgctctccaaaacctccttctggcgggccaagcgttcctccagctcttggactcttgtctgctcttcctctaatgcttccttcactctgttcttctcctgggtaatgcttttcgccaaagccttcttctgctgggccaggaggctctccagttcttgcattctcttccgttcttcctctaaagtctctttcgctctgtttctctcttgagtaatgtactcctccaaagccttaccgccttctcttccgtcagttgcctgattttggctttgagcttctcctcttgctctagcctctcctcgttcagcttctccttctctgccagatgctcccgcagcttttcctgcagtaaagactgctgagtttcctgagaactgttgaacttgatctttgttggggctggagggcaggatcccgaggtcccggaggagctgctccacctcctccagccaggacagcgcgtgcctcaggacgtccagcaccaccttctggagccccgagacaggtgggctcacctggaggtgctgaagaaggtcgacctccttcttcaggtcatggctgcaacaggatattttcatgcaagcctggcagctgtccagcgacgtcctcagcttctcgatgttctcggtggtctcctcctgcttggagttgctcagctgggtctctttctggagggtccactttttctgctgaaaattgatgttgtcctcagtgacctgggtaattttctctattaactgttggtcggtgacgggcttgtcccggaacggcttcgcccgtccataggtggccttgatgacttgacttctgaagtgctccagctgacctactgccctctccaaattgattttaatgacgctctctctgttccccatttcttgcagctgaagcaatttccttctggaatcctcctgaagcttctcttcaaccttgcttttttctctcagagtcctagagatcacgctttgttcagtacaactcttcctcagctctgccctaagcttcttcatttctttctccatgtcttggatttgggttttgcagagttttaactctttctcctgggcttccctgagctccctgtgagcatcttcctgttttaactcttcctttagcaccgagcatctagagccaagggcttccagctggtggtccttgtccttgttctgactttttaggtgactgacctcttcctttagttgttgaacttgctcatcctttgctaatatgtctttttgcaaagatgacaccatccctgatgtgatagcgttgtctctctttaagttctcgccctcattcttcagggatgtgatttctgagttccgctctgacagggtctggcacagcaccttgctgtagcctttctgtagggcactgatctggcttttcaagctctggatctctttctgtttggcatcgatgtcttcatccagaacctgacacttctgcgagatctccttctcattctgcctggaggtggtggtctctgacaccttctgactcagctcagccacttcattctgcaggtttgctattatgacgtctttgtatttggattcaatttcataatctgagagacggctgacctcttttcccagcagcagaattatttcatccttgtcctgctgggccaagtcctcctccacataaatctccgcagggggaactgccccaggaatcccctcggccactgatttttctgacagtttcatggcattggtccacacttgcttgatgacgggtggcttgcgggcgtcgtccaccacgaacgagaacatctccttgttggcgctcacaggccgcctgtgggaggccggcaggaccacggtgggtctgggaaaggcctgggaccagctcctttgcatcggtgctggctggacaccttggtggaaggggatatgtgatggtgggggggcctggtttggctgctgtgtggcacgaggtggctgtggccctggccatggtgctgggcccctcatccatgggaaagagaccggaggtggattttcaatgaccagttcataggtcagccctgcagacccaaatctcaggatgtctccagggatgagcttcacagccacgttttgaatgtggcactcgttgacaaacgtgccgttgcgggaattgaagtcctggagaacaaagctgcactccgcctcgttatattcaatgagtgcatggtggttgtcgatgtcaggagactgtaaaacaaggtctgaattttcatgccttccaattgtggtacttttatttaggacaaaaaagccttctgcgctctttagataggccttcatcctctctgttttccctggcgggaggaggaagcccacgctccgacctccgccgagagccctgccagctcgggaggcgtcgggccagctccggggcgaagcctcccggccgcgctcccgcggagtctccagctcgcacccggcaccccgcccgcccggccggcctgtgtacgcgcgttgccatggca

SEQ ID NO: 15960 - RNA, 724 nt, Homo sapiens
  source 1..724: mol_type = other RNA
gctgggattacaggcatgagccatcgcacccagccagggctgccaattcttttcaggaacgtgacaatctctgcagttgatagcgtcaccatagccaggggtatctaccactgtcaggcgtagcttgacccctcgctcttcaatttcaacagttgaagcctcaatctggacagttctttcaattttttctgctgctccaggtatgactctttctgggtacagatcagttaggaataggctgtttatgagagtcgattttcctagacctgattcaccgaccaccatcagtgtgaactcaaaaccttttttcactgattttcggtgaacttgattggggaggtttgcaaatccaacatagccaggtgtttctggatttataaactgagttggctgttgcttagacatcttttgtgaagcttcgtctctgctgccaaatgagttttggtgtccccattcctccagacaaaaaaaaaaaaaaaaatacccacaacttcttcttttacagcagtttctgtatgctcgctggtgcagaccttcgtcgcctctcctcgccgaaggtacccgcagacagggcctagtcgctctcccctcgcttatccacggcatccagccgatgggcttggaggtttgggggctggccagtcctccacgcccgccaaacagcccgagaacaggcgccgaccgaccgcgccgcggacccgcccagcgctcgcggtccgctcac

SEQ ID NO: 15961 - RNA, 642 nt, Homo sapiens
  source 1..642: mol_type = other RNA
gctgggattacaggcatgagccatcgcacccagccagggctgccaattcttttcaggaacgtgacaatctctgcagttgatagcgtcaccatagccaggggtatctaccactgtcaggcgtagcttgacccctcgctcttcaatttcaacagttgaagcctcaatctggacagttctttcaattttttctgctgctccaggtatgactctttctgggtacagatcagttaggaataggctgtttatgagagtcgattttcctagacctgattcaccttagacatcttttgtgaagcttcgtcttatgagctcggttttcttatgcttataagagtggaacaggtaatgagaatcttcgccttgcggtgggtaactggagtggggggaaggccgtttgttagaaggagacaagtgcccactgaggaggagagaggcggtcgcgggagggcaggtggtggcgggagtgcggagcgatcacggggagggggagccttcgcctctcctcctgtcctccaagaagatggcggcagcaccgagctggggcgccgagtacgactgggcgggggacggcgagcggccgcgcgaaactcgtctagcccaccaccgccgccgtctcgatgatcggggggcctctctgggatt

SEQ ID NO: 15962 - RNA, 6547 nt, Homo sapiens
  source 1..6547: mol_type = other RNA
gctgggattacaggcatgagccatcgcacccagcctcatttaacttttctgaatagactgtaagatcctcaaggggctccattttttaactaggtctttgtatttgtctgccactcaaacgtctgtttcagacatggagtcttgatacgttgcccaggttggccttgaatttctggtctcaggcgatcctcccacctcagcctcccaagtagatgggactacagatgcataccactatgcccggctttttttttttttttttttttttttttgaaatattaggttgctctggccgggcgcggtgactcacacctgcaatcccagcactttggaaggccaagacaggcagatcacaagatcaggagctcaagaccagcctggccaatatgctgaaatcccatctctactaaaaatacaaaaaaactcgctgggcatggtggcacatgcctgtaatcccagctactcggcagtctgaggcaggagaatcgcttgaacctgggaggcagaggttgcagtgagccgagatcacgccctgcactccagcctgggcaagaaaagaagcattagattgctctgttctgatgcctccagatcacatttgattacagcagttcttatttttcagacccacaaagaaaggacaggagagtcagatctgatcgtgggctaccatgtgataagaataaagaaatcaaccaatcagctttaagggaggcattttgggtcctggggctgtacaccttgccctggtactggagtaggtgagccctggatgagccacatggtgctggggcctctgaagaaagggctggggatgtgtttggaccaccacgaagggtacctggcccctcactctggcctctggaagcctggccaacatattcacaaaaagtaatgccccaagtcaggtgtttacactacatcaagtgtggggcagcgtgggggccaccaaggaatacggtgggcatgggcagcacggggccacactggcctggggccaactcctcatgggccatcctaggacccattctaatttcttaaaagagaaaatcttttaaaaaatgtttgcagaaacaagttggacctgaggccgcgcagagcctccccgacgggttcccaggagtggcgacagcatggagtccagtcagaagttcagtttgtccactctttattaaagccaggccctcctgctgacagctgcaggacagctgctggggcccaggagggacggagacagcagatcctggccatacagggctagagctgagattcccagagccccccaagcccaccttgcccttggccctttctgaggctcctgtcccgcagggagaggagaaacccagggccgaggtcattacccagcaccccaatgcctccctgggacccctgctctcctcaccaccccgccccgcaacctcaccaacctcacccagccaggctaactgaccgccaccacccaggccctcttcccacccaccaactaccgtgcctcctacccgcccccagccctggcagcctggctgctgcgctcagcccccaaggccatgtctacactaacgtggagggaactaggtctattagggaatgcagctgcaccaaaaatccgtttcctggccccattcacagtggccccaaaagcgtgaggggaatggggcttcacatgaactacaccccagctgcccgcccagtggcttccatgggcccagtccagagggtaggatgcccaccaggcaggggccttgcatagttgggtgcctggtttgtcactgagccacggctcaggtccacacccccccgaggtggacagccactgtgcaagctgccaggccacgggtgcctccactaaccaatttgtgaaatgggactctaaacagaaacactacttgttctagtgtaatgacagaagcagagttaaagggacctgcgagtgtcctagggccctgattatgggatgtggggaaagatccttcgaccaacctcagtcgctctaagtgagcgctgggctccgagaacggggcgtctgcctgctcccggagaggggcagcccagggaagtgaaagctggggctcagggctgcgagggcctcgggcgcccgtagatgtctgagtttgccacctccggctgagggagacgaaagtaccaaggactgagaggacaagcagagaccaaaaccgaaccggtgcggagggtgccggggtgacctcggtgcaagtgtgggtagagaagaggaggcggctcgagaataaggcttcaaactccctcaggaccctgtcaacacccgcgacccgtctgcctggccgtaagtttggtatctggctttttctcctcctagattcttcaggccatacaagaagtggaaataaatatccgcagacgacaagtttcaagttttcccactggagctccgccctttggaaacctacaaggcctcccctcgccgcgcgcagttaaaccttcgggacagactcggatgaccgggagggcccaagtctctcactgaggaatgggaagaagtggtcagccaaacccaccggcctcccaggcatcccgctggcccacctgggtggccgggcccctccctcgccgccacacccggttgcaaacacacaaatcccttgctccccagaccacccaagtcggaatccgagtgaaataaatagcatcgcccgccaactaccgccctgcttcacagcccgggcccacccaggggatatcgcagtctccgtgggggtgacgtcctggcctcgctgcctccgcgctgctcttctccccagagctcccccacgtctccggctgagcacacggacccggcgggcatgagacccggggccgcagggcgagggctgagggaaggcaccgcacccaggactgggaccctcagcctcccggggcccgaggagcggggggccggccgtccaagggaggggccggtggccctgcaggctgcgctgctgtcggccccgggcccctcacaggacgccctcccggtaggcgcccgagggcccggcgaacgcggcctggtgctcggagccgaagcttgtgccgcccgcgaactccagcagggcgctgccgcgctcaccggggccggcactggacggccccttggcggccgcctcgggcttgggcgcgggggctggggccgaacccgagcccggcgctgcggtggctccgcggtgcgtcttcatgtgggtgagcaagtgcgagctctgcgagaagcggcggccgcagttggcgcaggcgtagggccgctcgcccgtatgtgtgcgctggtgcgtgaccagcaccgagcgctgcgaaaagcgcttgccgcactcagggcacgggaaggggcgttcgcccgtgtggccgcgccggtgcttggccaggttggagcgctgcgcgaagccgcggccgcagtcggcgcagcggaagggcttctcgcccgtgtgcgtgcgccgatgccgcttgaagtccgagctgtggccgaagcccttgccgcagtcggggcagcggtgcggcttctcctcggcgtgcgcccactgatgccgcgtcagcgccgcgctctgcccgaagcgccggccgcactctccacacgcgtaaggccgctccccggtgtgcgcgcgcccgtgcgccgtcaagtgcgcgcgacggctgaaccccgcaccgcacacgccgcacacgaacggcttctcgcccgtgtggccgcgcacgtgcgccgccaagtgcgagccgcgggcgaaccgcgcgccgcactcggggcacgggaagggccgctcgccggtgtgtgtgcgccggtggcgcgccaggtgcgagccgtacacgaagctcttgccgcagtcggcgcagcgatgcggccgctcgcccgcgtggtagcgctggtgcttggccagcgcggcccggcgcccaaacgtcttgccgcagtccgagcagatccacgggctctcctcctccgccagcgcggccggcgcgggctccgccagcagacccccgatggcgggcccgaacgcgcgcaggccgcctccgccgcccgcggccccgccgccgccgaaagggtcgcacgccagcccggtaccctccaccagggagagcgggccccccaggggcgccgggagcgggcgcccgtcgaccggcagccgctctcggaagtcgggtaggcccaggatcgggaagctgtccgggtgcagccaggacttggggtgcacggggaagtggaagcccagcgggtgggaggaggggccttcgccctcccccaggccgttgcccagctccaggaagcgccgttccggcgcggggtccaccttgccgctgggggtgggcgccgccaccgccgcctcctctctctcctcggccgcggcctccgcctctccgtccgcctcgccaacttcagatccctctggcccagggtccgtgtcctcgggccccgcggcggccgccgtctcgccgggctcccgccgggggccgtcaccacccgcctccgcgcagcccccgccgcgtcggtggcgctggaagtcggcgcgcaggcggaaggcctggccgcagtcgggacagcagtgcgggcggtcggccgtgtgcaccgcctggtgccgtgccagcgccgagctctggctgaagctgcggccgcagtgcgaacacgggtagggtcgctcgccggtgtgcgtgcgctggtgcgtgaccaggtaggagcggcgcccgaagcccgcgccgcagaaggcgcagcggtagggccgctcgccagtatggatgcgtcggtgcgtaaccaggtgcgacttgtagacgaagcgcttgccgcagtccgggcacgggaagggcttctcgccggtgtgcgtgcgctggtggatggccaagtgcgagcggtacacgaagcccttgccgcactcctcgcagccgaagggcttgacggccgcgtggtagcgctggtgcttggccagccgcgagcggtgcgggaagaccttgccgcacacgtcgcacgtggtctccggcctcccggccggcggggccactgcggcggggaacgcccagggcgacagcaggttcgcacccggctcccggccgggcaggaaaggcttcgcttcagagccgtcggccaggacccccaggccgcctgggtcgggtccccacccctctggagtctgcgccgaatccgagtcgtcgggcccccacgtcccaggcacgtcccccacgccgtaggccgccgaccagagccctgggggctcgttctcctcctcggccacctccgccaggaagtcctcgtcgtcttcctcctcgtggtcctctatgtcgtccgtccagaaccaggctcctgtgtagacgccagtgacgatgtctccttcctcaggtcggggactatctgggacccaaggttcttccccttgttccagccggaagatcagatcgggcttgggaattgggtatcccaaggacacgagaatcccatagttctcctgcatgacttcctggtagaggccccgctggtctgcttccagcctttcccactcctccagggagaagtacacagccacatcttcaaacgtcaccagctcctgacacccagccgtcagcaaatcatcctcgtcctcatcctcctcctcctcttcctcctcctccaggtcctcatccctaggagtggctggagcccgggaggcctgcaggcccttttcctgaagaactggggacttggcatcaccaccacggctaagtcgctcctgggtccccaacgccggacactcctcctctgccagcacctccttcacatcctcctcctccacgtccgcctccacctccacctcggccaccgcctccacctgcgcatcctgcactacctctgccacaccctcctcctcctcctccaccactatctcctcctcctcttcttccacctcctgcacctcttcccccttttcctcctcctcctcctcttcttcctggtcagggtcgcactctgacccgtcctctgcccgctccagctgggcagctggggagtcgggagtcgtgtggagcgccgccatcctccctgggagcgagcctccacgtggcctggtcctcaacacacatgaaccaggccagcagggaacgccaagaggtctcagcacagacaggatgcaggcacttgcaaggcacaacggggctaggaggagagacaggtgccaggaagccggcaggtcaggcttcttccccagaagcagtggagagtctctgcctccaaagacgacactgagttctttctcccaagaagtccacccacggatgaccagagaaggtggaggaccagctcctgccggcagcagaagacagccgagcagcccaccggggctccttctgcagatgagggaaagcccggataaggcccccaaggtcacaaagcgggctcctggggcgacgggccgagcgcctcccgccccccagggggcgtccggagccgcctcctcctgcagagaccgcgcgggccgggctggccgagccacgggccggacaccggggccggggcctgcgggccggcggcggaccccgcgctacacaaagtgacggcccgggagctgcgcgacggcggcgcgtgggcaccggaagt

SEQ ID NO: 15963 - RNA, 4454 nt, Homo sapiens
  source 1..4454: mol_type = other RNA
gctgggattacaggcatgagccatcgcacccgtcctccagtaccattttaaacaaatacatattgtggactacgcaccaatagaaattaaggtggcaaaaccgtatcattagtaaagtaagtgaaagccttagtctttttgtttattccttattccccaaaggagttactaagtgaaggaattttccagctgcctttatttttttgagacggagtcttgttctgttgcccaggctggagtgcagtggcacgatcttggctcaccacaacctcctcctcctgggttccagcgattctcctgcctcagcctccagagtagctgggactacaggcgcccaccaacatgcccggctaatttgtgtatttacagtagagatggggtttcattatgttggccaggatggtcttgaactcctgacctcaagatcagcctgcctcggcctcccacagtgctgggattacatgcgtgagccactgcgcccggccttccagctgcatttctgaggtcacaagtatggccttaaatgattgccctcaagaacacagcttttgaaggtaatcatatgcaagtaaattacaatcaaatggaactgtatgattattttattattttaatgctaaactgaacagtgaactgaaatcagaggagaaagaaaatcaagctagtggctcactctcaatagtgtcctctaattttattgatgcttcagttttcataaagtgcaataaacaaaataaataaatgaaaaaagctttgaagatttatatacagttttgaggttaagataaattactgactatattcctttcagccttttaactctgtgaaagctgtaacgtacattaaaagcacattgaactaggttaaataatgatctttcccccttagatcaatctagtattaaggagtatataattatgcaagttcattctataacacaaggctagactaaaaggaaaatttttgtgctacagactaaatccagatacagtcaggtgctgagcagtattcctggcttcaaaataggaggtatctgtttcatcatctggctgggggatgaaaggcatagtctgatgctgcagattttcccagtccacatcactgaagagaggatgacgttttagctctcttttcagaatattctggaatacttgttgtggtgtttcatcattgaaagggggaattcctgttagaaattcaaacaagcaaactccaagtgcccaccagtctaccgcaggaccatgggccctgcctagtaacagctcaggtgcaaggtagtctggggttcctagaattcgcccatcatcaacgggggccacccctcttctcacactcttcggagttcggtatggagttcccgacttgatctgatttggggtctgctgatgtggcatacaggatcttcttttttgagtaggggttatagccatgggatatgaaccactgtaggcacacgaaatatccattgcatctaaagaagtcatgttcattctggatggttctgagttattggatgcattaatatgactgttaaaacttcgaaaagcaacagcatttcttttagaggctaacgttttcagcacctccaaaggaggacctaacattttttggttactctcttgtacagcagggttctcgacaccttttggtgaggtcttttcttggcaatctggtgttacaataagtggatcttcaatatttgattcttcaaaagaggattctttgatgcttctatctgaatctaagggctgactttctaatggactttccattatagaaattccaggaaaagatgaatcagagttcatagaaatatttttagaagctctatcatcatcagaacatagaaaactagaacttaagtagtccctcttactattcttttcacagtcttcatcgagttcacacataaggttttttgctatcattggtataggtaatttttctggtgtttgttgtttatcagtaaaagaattgacaatgttctccttattagcacagtcattttgttgacttttgtgcactgatagcttaaggtcctgcacttcaactgttaagcctgtattttgatttgtataacaatttgtcatttcgttatgcttatactctacacaagtttttttattctgtataatttttttacaaggactggagtcaaccaactcaaaatttctttttaaacttcttttcccaaggtgctcttcagatatcccaccagaatccacagcccactgatttgactgatggaaacctaactgacttgtgtcagtgtccatatttatattatttacatccagttctactgcttcccaagaaacttccccagagaagcattttttagcaaggtttacacaagagcgtccagtggtgggaagggcactgctgttatgaatgggagaaagagctaactccagatcctttttattgaaacctttcgtctcaatggcatttgcagattttgcgcataacttttcaactgcattccaactcatcattgttgggcccaatgcttcatcactttcctggcaatctttttcccatttgggactgctgtggcattctgattccacactggatatgaaggtgtgggattgactactggcactggatgtggccagccttttcctagactggagtaaattagaagttagacacttcacaggcattcctgggttggaggcaactgtttcaagacatgattttagtaatttgctagaataaggcgtagtgtccttttgatctacagacatagggcatacgagtccttgagaaagctgtgatgtttcagacagacaggctgaaaggatgtttgcagggtcttgatttttttctgcaattggtgtgttaaatcccaacgagctgataagcgataacacttgtcctggggttcttgaataatcttgtctaggttttgccattgatggtgttgtaaggatatccatcatattaatatctctattcaaagtaacttttgaaaggccaaaatccgtcagtttaatatgaccctcattagaaataagcatattgtccggtttcaagtccctgtggatgattccatgtctgtgaaggtagtctagagccagtgctacttcagaaatatatttcacagccatctcttcatcaaaataaccatatatatgtaggagagacttgacatctcccccaataagatattccattaccaagtagacattgtttgcagactgcagtgaataatacaaatggacaatgaatgggcttttgcttagtgccagtgcatctctctcagcttggacctgatgagtcatatttttgttgatcatgtctgcttttttaacaacctttactgcatacaatttgccgcctttctgccccagatacactttcccgaaggcgccccggctaatgggcttcactatgctgaattcctcaatggagggcggttttggcactgcgatcctattcacgccctcctcagtcgccgcgcctcctccaggctccttcttgcttcccgcggtgggatccatcgctggacagcatacagcggccccgcagacactgcccctccgcgagcagccactcccgccaactgggttcaaagtgaggctccgcccacgccgcgcgcggccgtgacgtcaccccgccgccgcgccccgccctcgtcacctcccctacgcagacgcggacggagggggcgtcgggaaagccccgacttcgcagccttacactcttcgtgggcggcgaccgcggccccactgacatcattcctcatgagggaggaggcacaaacagttctgggccgaccagaaaaaggacgactgggacttgactctgaatcgcaggatttgaagagatttctcctggcttcccaacgaggctggtgggaagcggtcctcctcccatacacgacctcccaccctcgcgaggcgtagaaaccagttctgactgtacagtaaagcgagggccagggctgaggtctggaagctaatgaaagcacagaaagtgtcgaaactggatgagcaggaagcgagtggcctcccctgtcatctgacgttttcccaggatgtaatttgcctgactgaaacagatcaggaccaacagggagagttttcgatttagtgtgaggaaaagagcactaaattgtagcaaaagaccttattgctcaaggcccagtcagaagatttcataaggaagctgtagaaagtcttaagaggaaatcagccgggcgtggtggcgggcacctgtaatcccagctactcgggaggctgaggcaggagaatcgcttgaacccggggagcagaggttgcagtgagccgagatcgcgccactgtacgccagcctgggcgaaagaacgaaactccgtctccaaaaaaaaaaaaaacgaagaaaaagtccaaagagggtaaaggctgttctccccttaaaaaacagctaaagacctttgggggcgctgctccttgtaaatgtcaactact

SEQ ID NO: 15964 - RNA, 4469 nt, Homo sapiens
  source 1..4469: mol_type = other RNA
gctgggattacaggcatgagccatcgcacccgtcctccagtaccattttaaacaaatacatattgtggactacgcaccaatagaaattaaggtggcaaaaccgtatcattagtaaagtaagtgaaagccttagtctttttgtttattccttattccccaaaggagttactaagtgaaggaattttccagctgcctttatttttttgagacggagtcttgttctgttgcccaggctggagtgcagtggcacgatcttggctcaccacaacctcctcctcctgggttccagcgattctcctgcctcagcctccagagtagctgggactacaggcgcccaccaacatgcccggctaatttgtgtatttacagtagagatggggtttcattatgttggccaggatggtcttgaactcctgacctcaagatcagcctgcctcggcctcccacagtgctgggattacatgcgtgagccactgcgcccggccttccagctgcatttctgaggtcacaagtatggccttaaatgattgccctcaagaacacagcttttgaaggtaatcatatgcaagtaaattacaatcaaatggaactgtatgattattttattattttaatgctaaactgaacagtgaactgaaatcagaggagaaagaaaatcaagctagtggctcactctcaatagtgtcctctaattttattgatgcttcagttttcataaagtgcaataaacaaaataaataaatgaaaaaagctttgaagatttatatacagttttgaggttaagataaattactgactatattcctttcagccttttaactctgtgaaagctgtaacgtacattaaaagcacattgaactaggttaaataatgatctttcccccttagatcaatctagtattaaggagtatataattatgcaagttcattctataacacaaggctagactaaaaggaaaatttttgtgctacagactaaatccagatacagtcaggtgctgagcagtattcctggcttcaaaataggaggtatctgtttcatcatctggctgggggatgaaaggcatagtctgatgctgcagattttcccagtccacatcactgaagagaggatgacgttttagctctcttttcagaatattctggaatacttgttgtggtgtttcatcattgaaagggggaattcctgttagaaattcaaacaagcaaactccaagtgcccaccagtctaccgcaggaccggaagtcagaaatccatgggccctgcctagtaacagctcaggtgcaaggtagtctggggttcctagaattcgcccatcatcaacgggggccacccctcttctcacactcttcggagttcggtatggagttcccgacttgatctgatttggggtctgctgatgtggcatacaggatcttcttttttgagtaggggttatagccatgggatatgaaccactgtaggcacacgaaatatccattgcatctaaagaagtcatgttcattctggatggttctgagttattggatgcattaatatgactgttaaaacttcgaaaagcaacagcatttcttttagaggctaacgttttcagcacctccaaaggaggacctaacattttttggttactctcttgtacagcagggttctcgacaccttttggtgaggtcttttcttggcaatctggtgttacaataagtggatcttcaatatttgattcttcaaaagaggattctttgatgcttctatctgaatctaagggctgactttctaatggactttccattatagaaattccaggaaaagatgaatcagagttcatagaaatatttttagaagctctatcatcatcagaacatagaaaactagaacttaagtagtccctcttactattcttttcacagtcttcatcgagttcacacataaggttttttgctatcattggtataggtaatttttctggtgtttgttgtttatcagtaaaagaattgacaatgttctccttattagcacagtcattttgttgacttttgtgcactgatagcttaaggtcctgcacttcaactgttaagcctgtattttgatttgtataacaatttgtcatttcgttatgcttatactctacacaagtttttttattctgtataatttttttacaaggactggagtcaaccaactcaaaatttctttttaaacttcttttcccaaggtgctcttcagatatcccaccagaatccacagcccactgatttgactgatggaaacctaactgacttgtgtcagtgtccatatttatattatttacatccagttctactgcttcccaagaaacttccccagagaagcattttttagcaaggtttacacaagagcgtccagtggtgggaagggcactgctgttatgaatgggagaaagagctaactccagatcctttttattgaaacctttcgtctcaatggcatttgcagattttgcgcataacttttcaactgcattccaactcatcattgttgggcccaatgcttcatcactttcctggcaatctttttcccatttgggactgctgtggcattctgattccacactggatatgaaggtgtgggattgactactggcactggatgtggccagccttttcctagactggagtaaattagaagttagacacttcacaggcattcctgggttggaggcaactgtttcaagacatgattttagtaatttgctagaataaggcgtagtgtccttttgatctacagacatagggcatacgagtccttgagaaagctgtgatgtttcagacagacaggctgaaaggatgtttgcagggtcttgatttttttctgcaattggtgtgttaaatcccaacgagctgataagcgataacacttgtcctggggttcttgaataatcttgtctaggttttgccattgatggtgttgtaaggatatccatcatattaatatctctattcaaagtaacttttgaaaggccaaaatccgtcagtttaatatgaccctcattagaaataagcatattgtccggtttcaagtccctgtggatgattccatgtctgtgaaggtagtctagagccagtgctacttcagaaatatatttcacagccatctcttcatcaaaataaccatatatatgtaggagagacttgacatctcccccaataagatattccattaccaagtagacattgtttgcagactgcagtgaataatacaaatggacaatgaatgggcttttgcttagtgccagtgcatctctctcagcttggacctgatgagtcatatttttgttgatcatgtctgcttttttaacaacctttactgcatacaatttgccgcctttctgccccagatacactttcccgaaggcgccccggctaatgggcttcactatgctgaattcctcaatggagggcggttttggcactgcgatcctattcacgccctcctcagtcgccgcgcctcctccaggctccttcttgcttcccgcggtgggatccatcgctggacagcatacagcggccccgcagacactgcccctccgcgagcagccactcccgccaactgggttcaaagtgaggctccgcccacgccgcgcgcggccgtgacgtcaccccgccgccgcgccccgccctcgtcacctcccctacgcagacgcggacggagggggcgtcgggaaagccccgacttcgcagccttacactcttcgtgggcggcgaccgcggccccactgacatcattcctcatgagggaggaggcacaaacagttctgggccgaccagaaaaaggacgactgggacttgactctgaatcgcaggatttgaagagatttctcctggcttcccaacgaggctggtgggaagcggtcctcctcccatacacgacctcccaccctcgcgaggcgtagaaaccagttctgactgtacagtaaagcgagggccagggctgaggtctggaagctaatgaaagcacagaaagtgtcgaaactggatgagcaggaagcgagtggcctcccctgtcatctgacgttttcccaggatgtaatttgcctgactgaaacagatcaggaccaacagggagagttttcgatttagtgtgaggaaaagagcactaaattgtagcaaaagaccttattgctcaaggcccagtcagaagatttcataaggaagctgtagaaagtcttaagaggaaatcagccgggcgtggtggcgggcacctgtaatcccagctactcgggaggctgaggcaggagaatcgcttgaacccggggagcagaggttgcagtgagccgagatcgcgccactgtacgccagcctgggcgaaagaacgaaactccgtctccaaaaaaaaaaaaaacgaagaaaaagtccaaagagggtaaaggctgttctccccttaaaaaacagctaaagacctttgggggcgctgctccttgtaaatgtcaactact

SEQ ID NO: 15965 - RNA, 3566 nt, Homo sapiens
  source 1..3566: mol_type = other RNA
gctgggattacaggcatgagccatcgcacccgtcctccagtaccattttaaacaaatacatattgtggactacgcaccaatagaaattaaggtggcaaaaccgtatcattagtaaagtaagtgaaagccttagtctttttgtttattccttattccccaaaggagttactaagtgaaggaattttccagctgcctttatttttttgagacggagtcttgttctgttgcccaggctggagtgcagtggcacgatcttggctcaccacaacctcctcctcctgggttccagcgattctcctgcctcagcctccagagtagctgggactacaggcgcccaccaacatgcccggctaatttgtgtatttacagtagagatggggtttcattatgttggccaggatggtcttgaactcctgacctcaagatcagcctgcctcggcctcccacagtgctgggattacatgcgtgagccactgcgcccggccttccagctgcatttctgaggtcacaagtatggccttaaatgattgccctcaagaacacagcttttgaaggtaatcatatgcaagtaaattacaatcaaatggaactgtatgattattttattattttaatgctaaactgaacagtgaactgaaatcagaggagaaagaaaatcaagctagtggctcactctcaatagtgtcctctaattttattgatgcttcagttttcataaagtgcaataaacaaaataaataaatgaaaaaagctttgaagatttatatacagttttgaggttaagataaattactgactatattcctttcagccttttaactctgtgaaagctgtaacgtacattaaaagcacattgaactaggttaaataatgatctttcccccttagatcaatctagtattaaggagtatataattatgcaagttcattctataacacaaggctagactaaaaggaaaatttttgtgctacagactaaatccagatacagtcaggtgctgagcagtattcctggcttcaaaataggaggtatctgtttcatcatctggctgggggatgaaaggcatagtctgatgctgcagattttcccagtccacatcactgaagagaggatgacgttttagctctttcattccagctctctttgtatcatcaatggttaaaagtatttctactgcactttgagcattatcagataacttttcttcaccttctggccaagggatatcatgggccctgcctagtaacagctcaggtgcaaggtagtctggggttcctagaattcgcccatcatcaacgggggccacccctcttctcacactcttcggagttcggtatggagttcccgacttgatctgatttggggtctgatgtggcatacaggatcttcttttttgagtaggggttatagccatgggatatgaaccactgtaggcacacgaaatatccattgcatctaaagaagtcatgttcattctggatggttctgagttattggatgcattaatatgactgttaaaacttcgaaaagcaacagcatttcttttagaggctaacgttttcagcacctccaaaggaggacctaacattttttggttactctcttgtacagcagggttctcgacaccttttggtgaggtcttttcttggcaatctggtgttacaataagtggatcttcaatatttgattcttcaaaagaggattctttgatgcttctatctgaatctaagggctgactttctaatggactttccattatagaaattccaggaaaagatgaatcagagttcatagaaatatttttagaagctctatcatcatcagaacatagaaaactagaacttaagtagtccctcttactattcttttcacagtcttcatcgagttcacacataaggttttttgctatcattggtataggtaatttttctggtgtttgttgtttatcagtaaaagaattgacaatgttctccttattagcacagtcattttgttgacttttgtgcactgatagcttaaggtcctgcacttcaactgttaagcctgtattttgatttgtataacaatttgtcatttcgttatgcttatactctacacaagtttttttattctgtataatttttttacaaggactggagtcaaccaactcaaaatttctttttaaacttcttttcccaaggtgctcttcagatatcccaccagaatccacagcccactgatttgactgatggaaacctaactgacttgtgtcagtgtccatatttatattatttacatccagttctactgcttcccaagaaacttccccagagaagcattttttagcaaggtttacacaagagcgtccagtggtgggaagggcactgctgttatgaatgggagaaagagctaactccagatcctttttattgaaacctttcgtctcaatggcatttgcagattttgcgcataacttttcaactgcattccaactcatcattgttgggcccaatgcttcatcactttcctggcaatctttttcccatttgggactgctgtggcattctgattccacactggatatgaaggtgtgggattgactactggcactggatgtggccagccttttcctagactggagtaaattagaagttagacacttcacaggcattcctgggttggaggcaactgtttcaagacatgattttagtaatttgctagaataaggcgtagtgtccttttgatctacagacatagggcatacgagtccttgagaaagctgtgatgtttcagacagacaggctgaaaggatgtttgcagggtcttgatttttttctgcaattggtgtgttaaatcccaacgagctgataagcgataacacttgtcctggggttcttgaataatcttgtctaggttttgccattgatggtgttgtaaggatatccatcatattaatatctctattcaaagtaacttttgaaaggccaaaatccgtcagtttaatatgaccctcattagaaataagcatattgtccggtttcaagtccctgtggatgattccatgtctgtgaaggtagtctagagccagtgctacttcagaaatatatttcacagccatctcttcatcaaaataaccatatatatgtaggagagacttgacatctcccccaataagatattccattaccaagtagacattgtttgcagactgcagtgaataatacaaatggacaatgaatgggcttttgcttagtgccagtgcatctctctcagcttggacctgatgagtcatatttttgttgatcatgtctgcttttttaacaacctttactgcatacaatttgccgcctttctgccccagatacactttcccgaaggcgccccggctaatgggcttcactatgctgaattcctcaatggagggcggttttggcactgcgatcctattcacgccctcctcagtcgccgcgcctcctccaggctccttcttgcttcccgcggtgggatccatcgctggacagcatacagcggccccgcagacactgcccctccgcgagcagccactcccgccaactgggttcaaagt

SEQ ID NO: 15966 - RNA, 4442 nt, Homo sapiens
  source 1..4442: mol_type = other RNA
gctgggattacaggcatgagccatcgcacccgtcctccagtaccattttaaacaaatacatattgtggactacgcaccaatagaaattaaggtggcaaaaccgtatcattagtaaagtaagtgaaagccttagtctttttgtttattccttattccccaaaggagttactaagtgaaggaattttccagctgcctttatttttttgagacggagtcttgttctgttgcccaggctggagtgcagtggcacgatcttggctcaccacaacctcctcctcctgggttccagcgattctcctgcctcagcctccagagtagctgggactacaggcgcccaccaacatgcccggctaatttgtgtatttacagtagagatggggtttcattatgttggccaggatggtcttgaactcctgacctcaagatcagcctgcctcggcctcccacagtgctgggattacatgcgtgagccactgcgcccggccttccagctgcatttctgaggtcacaagtatggccttaaatgattgccctcaagaacacagcttttgaaggtaatcatatgcaagtaaattacaatcaaatggaactgtatgattattttattattttaatgctaaactgaacagtgaactgaaatcagaggagaaagaaaatcaagctagtggctcactctcaatagtgtcctctaattttattgatgcttcagttttcataaagtgcaataaacaaaataaataaatgaaaaaagctttgaagatttatatacagttttgaggttaagataaattactgactatattcctttcagccttttaactctgtgaaagctgtaacgtacattaaaagcacattgaactaggttaaataatgatctttcccccttagatcaatctagtattaaggagtatataattatgcaagttcattctataacacaaggctagactaaaaggaaaatttttgtgctacagactaaatccagatacagtcaggtgctgagcagtattcctggcttcaaaataggaggtatctgtttcatcatctggctgggggatgaaaggcatagtctgatgctgcagattttcccagtccacatcactgaagagaggatgacgttttagctctttcattccagctctctttgtatcatcaatggttaaaagtatttctactgcactttgagcattatcagataacttttcttcaccttctggccaagggatatcatgggccctgcctagtaacagctcaggtgcaaggtagtctggggttcctagaattcgcccatcatcaacgggggccacccctcttctcacactcttcggagttcggtatggagttcccgacttgatctgatttggggtctgctgatgtggcatacaggatcttcttttttgagtaggggttatagccatgggatatgaaccactgtaggcacacgaaatatccattgcatctaaagaagtcatgttcattctggatggttctgagttattggatgcattaatatgactgttaaaacttcgaaaagcaacagcatttcttttagaggctaacgttttcagcacctccaaaggaggacctaacattttttggttactctcttgtacagcagggttctcgacaccttttggtgaggtcttttcttggcaatctggtgttacaataagtggatcttcaatatttgattcttcaaaagaggattctttgatgcttctatctgaatctaagggctgactttctaatggactttccattatagaaattccaggaaaagatgaatcagagttcatagaaatatttttagaagctctatcatcatcagaacatagaaaactagaacttaagtagtccctcttactattcttttcacagtcttcatcgagttcacacataaggttttttgctatcattggtataggtaatttttctggtgtttgttgtttatcagtaaaagaattgacaatgttctccttattagcacagtcattttgttgacttttgtgcactgatagcttaaggtcctgcacttcaactgttaagcctgtattttgatttgtataacaatttgtcatttcgttatgcttatactctacacaagtttttttattctgtataatttttttacaaggactggagtcaaccaactcaaaatttctttttaaacttcttttcccaaggtgctcttcagatatcccaccagaatccacagcccactgatttgactgatggaaacctaactgacttgtgtcagtgtccatatttatattatttacatccagttctactgcttcccaagaaacttccccagagaagcattttttagcaaggtttacacaagagcgtccagtggtgggaagggcactgctgttatgaatgggagaaagagctaactccagatcctttttattgaaacctttcgtctcaatggcatttgcagattttgcgcataacttttcaactgcattccaactcatcattgttgggcccaatgcttcatcactttcctggcaatctttttcccatttgggactgctgtggcattctgattccacactggatatgaaggtgtgggattgactactggcactggatgtggccagccttttcctagactggagtaaattagaagttagacacttcacaggcattcctgggttggaggcaactgtttcaagacatgattttagtaatttgctagaataaggcgtagtgtccttttgatctacagacatagggcatacgagtccttgagaaagctgtgatgtttcagacagacaggctgaaaggatgtttgcagggtcttgatttttttctgcaattggtgtgttaaatcccaacgagctgataagcgataacacttgtcctggggttcttgaataatcttgtctaggttttgccattgatggtgttgtaaggatatccatcatattaatatctctattcaaagtaacttttgaaaggccaaaatccgtcagtttaatatgaccctcattagaaataagcatattgtccggtttcaagtccctgtggatgattccatgtctgtgaaggtagtctagagccagtgctacttcagaaatatatttcacagccatctcttcatcaaaataaccatatatatgtaggagagacttgacatctcccccaataagatattccattaccaagtagacattgtttgcagactgcagtgaataatacaaatggacaatgaatgggcttttgcttagtgccagtgcatctctctcagcttggacctgatgagtcatatttttgttgatcatgtctgcttttttaacaacctttactgcatacaatttgccgcctttctgccccagatacactttcccgaaggcgccccggctaatgggcttcactatgctgaattcctcaatggagggcggttttggcactgcgatcctattcacgccctcctcagtcgccgcgcctcctccaggctccttcttgcttcccgcggtgggatccatcgctggacagcatacagcggccccgcagacactgcccctccgcgagcagccactcccgccaactgggttcaaagtgaggctccgcccacgccgcgcgcggccgtgacgtcaccccgccgccgcgccccgccctcgtcacctcccctacgcagacgcggacggagggggcgtcgggaaagccccgacttcgcagccttacactcttcgtgggcggcgaccgcggccccactgacatcattcctcatgagggaggaggcacaaacagttctgggccgaccagaaaaaggacgactgggacttgactctgaatcgcaggatttgaagagatttctcctggcttcccaacgaggctggtgggaagcggtcctcctcccatacacgacctcccaccctcgcgaggcgtagaaaccagttctgactgtacagtaaagcgagggccagggctgaggtctggaagctaatgaaagcacagaaagtgtcgaaactggatgagcaggaagcgagtggcctcccctgtcatctgacgttttcccaggatgtaatttgcctgactgaaacagatcaggaccaacagggagagttttcgatttagtgtgaggaaaagagcactaaattgtagcaaaagaccttattgctcaaggcccagtcagaagatttcataaggaagctgtagaaagtcttaagaggaaatcagccgggcgtggtggcgggcacctgtaatcccagctactcgggaggctgaggcaggagaatcgcttgaacccggggagcagaggttgcagtgagccgagatcgcgccactgtacgccagcctgggcgaaagaacgaaactccgtctccaaaaaaaaaaaaaacgaagaaaaagtccaaagagggtaaaggctgttctccccttaaaaaacagctaaagacctttgggggcgctgctccttgtaaatgtcaactact

SEQ ID NO: 15967 - RNA, 3680 nt, Homo sapiens
  source 1..3680: mol_type = other RNA
gctgggattacaggcatgagccatcgcacccgtcctccagtaccattttaaacaaatacatattgtggactacgcaccaatagaaattaaggtggcaaaaccgtatcattagtaaagtaagtgaaagccttagtctttttgtttattccttattccccaaaggagttactaagtgaaggaattttccagctgcctttatttttttgagacggagtcttgttctgttgcccaggctggagtgcagtggcacgatcttggctcaccacaacctcctcctcctgggttccagcgattctcctgcctcagcctccagagtagctgggactacaggcgcccaccaacatgcccggctaatttgtgtatttacagtagagatggggtttcattatgttggccaggatggtcttgaactcctgacctcaagatcagcctgcctcggcctcccacagtgctgggattacatgcgtgagccactgcgcccggccttccagctgcatttctgaggtcacaagtatggccttaaatgattgccctcaagaacacagcttttgaaggtaatcatatgcaagtaaattacaatcaaatggaactgtatgattattttattattttaatgctaaactgaacagtgaactgaaatcagaggagaaagaaaatcaagctagtggctcactctcaatagtgtcctctaattttattgatgcttcagttttcataaagtgcaataaacaaaataaataaatgaaaaaagctttgaagatttatatacagttttgaggttaagataaattactgactatattcctttcagccttttaactctgtgaaagctgtaacgtacattaaaagcacattgaactaggttaaataatgatctttcccccttagatcaatctagtattaaggagtatataattatgcaagttcattctataacacaaggctagactaaaaggaaaatttttgtgctacagactaaatccagatacagtcaggtgctgagcagtattcctggcttcaaaataggaggtatctgtttcatcatctggctgggggatgaaaggcatagtctgatgctgcagattttcccagtccacatcactgaagagaggatgacgttttagctctttcattccagctctctttgtatcatcaatggttaaaagtatttctactgcactttgagcattatcagataacttttcttcaccttctggccaagggatatctcttttcagaatattctggaatacttgttgtggtgtttcatcattgaaagggggaattcctgttagaaattcaaacaagcaaactccaagtgcccaccagtctaccgcaggaccatgggccctgcctagtaacagctcaggtgcaaggtagtctggggttcctagaattcgcccatcatcaacgggggccacccctcttctcacactcttcggagttcggtatggagttcccgacttgatctgatttggggtctgatgtggcatacaggatcttcttttttgagtaggggttatagccatgggatatgaaccactgtaggcacacgaaatatccattgcatctaaagaagtcatgttcattctggatggttctgagttattggatgcattaatatgactgttaaaacttcgaaaagcaacagcatttcttttagaggctaacgttttcagcacctccaaaggaggacctaacattttttggttactctcttgtacagcagggttctcgacaccttttggtgaggtcttttcttggcaatctggtgttacaataagtggatcttcaatatttgattcttcaaaagaggattctttgatgcttctatctgaatctaagggctgactttctaatggactttccattatagaaattccaggaaaagatgaatcagagttcatagaaatatttttagaagctctatcatcatcagaacatagaaaactagaacttaagtagtccctcttactattcttttcacagtcttcatcgagttcacacataaggttttttgctatcattggtataggtaatttttctggtgtttgttgtttatcagtaaaagaattgacaatgttctccttattagcacagtcattttgttgacttttgtgcactgatagcttaaggtcctgcacttcaactgttaagcctgtattttgatttgtataacaatttgtcatttcgttatgcttatactctacacaagtttttttattctgtataatttttttacaaggactggagtcaaccaactcaaaatttctttttaaacttcttttcccaaggtgctcttcagatatcccaccagaatccacagcccactgatttgactgatggaaacctaactgacttgtgtcagtgtccatatttatattatttacatccagttctactgcttcccaagaaacttccccagagaagcattttttagcaaggtttacacaagagcgtccagtggtgggaagggcactgctgttatgaatgggagaaagagctaactccagatcctttttattgaaacctttcgtctcaatggcatttgcagattttgcgcataacttttcaactgcattccaactcatcattgttgggcccaatgcttcatcactttcctggcaatctttttcccatttgggactgctgtggcattctgattccacactggatatgaaggtgtgggattgactactggcactggatgtggccagccttttcctagactggagtaaattagaagttagacacttcacaggcattcctgggttggaggcaactgtttcaagacatgattttagtaatttgctagaataaggcgtagtgtccttttgatctacagacatagggcatacgagtccttgagaaagctgtgatgtttcagacagacaggctgaaaggatgtttgcagggtcttgatttttttctgcaattggtgtgttaaatcccaacgagctgataagcgataacacttgtcctggggttcttgaataatcttgtctaggttttgccattgatggtgttgtaaggatatccatcatattaatatctctattcaaagtaacttttgaaaggccaaaatccgtcagtttaatatgaccctcattagaaataagcatattgtccggtttcaagtccctgtggatgattccatgtctgtgaaggtagtctagagccagtgctacttcagaaatatatttcacagccatctcttcatcaaaataaccatatatatgtaggagagacttgacatctcccccaataagatattccattaccaagtagacattgtttgcagactgcagtgaataatacaaatggacaatgaatgggcttttgcttagtgccagtgcatctctctcagcttggacctgatgagtcatatttttgttgatcatgtctgcttttttaacaacctttactgcatacaatttgccgcctttctgccccagatacactttcccgaaggcgccccggctaatgggcttcactatgctgaattcctcaatggagggcggttttggcactgcgatcctattcacgccctcctcagtcgccgcgcctcctccaggctccttcttgcttcccgcggtgggatccatcgctggacagcatacagcggccccgcagacactgcccctccgcgagcagccactcccgccaactgggttcaaagt

SEQ ID NO: 15968 - RNA, 3803 nt, Homo sapiens
  source 1..3803: mol_type = other RNA
gctgggattacaggcatgagccatcgcacccgtcctccagtaccattttaaacaaatacatattgtggactacgcaccaatagaaattaaggtggcaaaaccgtatcattagtaaagtaagtgaaagccttagtctttttgtttattccttattccccaaaggagttactaagtgaaggaattttccagctgcctttatttttttgagacggagtcttgttctgttgcccaggctggagtgcagtggcacgatcttggctcaccacaacctcctcctcctgggttccagcgattctcctgcctcagcctccagagtagctgggactacaggcgcccaccaacatgcccggctaatttgtgtatttacagtagagatggggtttcattatgttggccaggatggtcttgaactcctgacctcaagatcagcctgcctcggcctcccacagtgctgggattacatgcgtgagccactgcgcccggccttccagctgcatttctgaggtcacaagtatggccttaaatgattgccctcaagaacacagcttttgaaggtaatcatatgcaagtaaattacaatcaaatggaactgtatgattattttattattttaatgctaaactgaacagtgaactgaaatcagaggagaaagaaaatcaagctagtggctcactctcaatagtgtcctctaattttattgatgcttcagttttcataaagtgcaataaacaaaataaataaatgaaaaaagctttgaagatttatatacagttttgaggttaagataaattactgactatattcctttcagccttttaactctgtgaaagctgtaacgtacattaaaagcacattgaactaggttaaataatgatctttcccccttagatcaatctagtattaaggagtatataattatgcaagttcattctataacacaaggctagactaaaaggaaaatttttgtgctacagactaaatccagatacagtcaggtgctgagcagtattcctggcttcaaaataggaggtatctgtttcatcatctggctgggggatgaaaggcatagtctgatgctgcagattttcccagtccacatcactgaagagaggatgacgttttagctctttcattccagctctctttgtatcatcaatggttaaaagtatttctactgcactttgagcattatcagataacttttcttcaccttctggccaagggatatctcttttcagaatattctggaatacttgttgtggtgtttcatcattgaaagggggaattcctgttagaaattcaaacaagcaaactccaagtgcccaccagtctaccgcaggaccatgggccctgcctagtaacagctcaggtgcaaggtagtctggggttcctagaattcgcccatcatcaacgggggccacccctcttctcacactcttcggagttcggtatggagttcccgacttgatctgatttggggtctgctgatgtggcatacaggatcttcttttttgagtaggggttatagccatgggatatgaaccactgtaggcacacgaaatatccattgcatctaaagaagtcatgttcattctggatggttctgagttattggatgcattaatatgactgttaaaacttcgaaaagcaacagcatttcttttagaggctaacgttttcagcacctccaaaggaggacctaacattttttggttactctcttgtacagcagggttctcgacaccttttggtgaggtcttttcttggcaatctggtgttacaataagtggatcttcaatatttgattcttcaaaagaggattctttgatgcttctatctgaatctaagggctgactttctaatggactttccattatagaaattccaggaaaagatgaatcagagttcatagaaatatttttagaagctctatcatcatcagaacatagaaaactagaacttaagtagtccctcttactattcttttcacagtcttcatcgagttcacacataaggttttttgctatcattggtataggtaatttttctggtgtttgttgtttatcagtaaaagaattgacaatgttctccttattagcacagtcattttgttgacttttgtgcactgatagcttaaggtcctgcacttcaactgttaagcctgtattttgatttgtataacaatttgtcatttcgttatgcttatactctacacaagtttttttattctgtataatttttttacaaggactggagtcaaccaactcaaaatttctttttaaacttcttttcccaaggtgctcttcagatatcccaccagaatccacagcccactgatttgactgatggaaacctaactgacttgtgtcagtgtccatatttatattatttacatccagttctactgcttcccaagaaacttccccagagaagcattttttagcaaggtttacacaagagcgtccagtggtgggaagggcactgctgttatgaatgggagaaagagctaactccagatcctttttattgaaacctttcgtctcaatggcatttgcagattttgcgcataacttttcaactgcattccaactcatcattgttgggcccaatgcttcatcactttcctggcaatctttttcccatttgggactgctgtggcattctgattccacactggatatgaaggtgtgggattgactactggcactggatgtggccagccttttcctagactggagtaaattagaagttagacacttcacaggcattcctgggttggaggcaactgtttcaagacatgattttagtaatttgctagaataaggcgtagtgtccttttgatctacagacatagggcatacgagtccttgagaaagctgtgatgtttcagacagacaggctgaaaggatgtttgcagggtcttgatttttttctgcaattggtgtgttaaatcccaacgagctgataagcgataacacttgtcctggggttcttgaataatcttgtctaggttttgccattgatggtgttgtaaggatatccatcatattaatatctctattcaaagtaacttttgaaaggccaaaatccgtcagtttaatatgaccctcattagaaataagcatattgtccggtttcaagtccctctactcccagacacttgggaggctaaggcagggggattgcttgagccccagaggtcgaggctgcagtgagccaaggtcaagtcactgcactgcacaacctggatgacaaagtgagaccctgtggatgattccatgtctgtgaaggtagtctagagccagtgctacttcagaaatatatttcacagccatctcttcatcaaaataaccatatatatgtaggagagacttgacatctcccccaataagatattccattaccaagtagacattgtttgcagactgcagtgaataatacaaatggacaatgaatgggcttttgcttagtgccagtgcatctctctcagcttggacctgatgagtcatatttttgttgatcatgtctgcttttttaacaacctttactgcatacaatttgccgcctttctgccccagatacactttcccgaaggcgccccggctaatgggcttcactatgctgaattcctcaatggagggcggttttggcactgcgatcctattcacgccctcctcagtcgccgcgcctcctccaggctccttcttgcttcccgcggtgggatccatcgctggacagcatacagcggccccgcagacactgcccctccgcgagcagccactcccgccaactgggttcaaagt

SEQ ID NO: 15969 - RNA, 3683 nt, Homo sapiens
  source 1..3683: mol_type = other RNA
gctgggattacaggcatgagccatcgcacccgtcctccagtaccattttaaacaaatacatattgtggactacgcaccaatagaaattaaggtggcaaaaccgtatcattagtaaagtaagtgaaagccttagtctttttgtttattccttattccccaaaggagttactaagtgaaggaattttccagctgcctttatttttttgagacggagtcttgttctgttgcccaggctggagtgcagtggcacgatcttggctcaccacaacctcctcctcctgggttccagcgattctcctgcctcagcctccagagtagctgggactacaggcgcccaccaacatgcccggctaatttgtgtatttacagtagagatggggtttcattatgttggccaggatggtcttgaactcctgacctcaagatcagcctgcctcggcctcccacagtgctgggattacatgcgtgagccactgcgcccggccttccagctgcatttctgaggtcacaagtatggccttaaatgattgccctcaagaacacagcttttgaaggtaatcatatgcaagtaaattacaatcaaatggaactgtatgattattttattattttaatgctaaactgaacagtgaactgaaatcagaggagaaagaaaatcaagctagtggctcactctcaatagtgtcctctaattttattgatgcttcagttttcataaagtgcaataaacaaaataaataaatgaaaaaagctttgaagatttatatacagttttgaggttaagataaattactgactatattcctttcagccttttaactctgtgaaagctgtaacgtacattaaaagcacattgaactaggttaaataatgatctttcccccttagatcaatctagtattaaggagtatataattatgcaagttcattctataacacaaggctagactaaaaggaaaatttttgtgctacagactaaatccagatacagtcaggtgctgagcagtattcctggcttcaaaataggaggtatctgtttcatcatctggctgggggatgaaaggcatagtctgatgctgcagattttcccagtccacatcactgaagagaggatgacgttttagctctttcattccagctctctttgtatcatcaatggttaaaagtatttctactgcactttgagcattatcagataacttttcttcaccttctggccaagggatatctcttttcagaatattctggaatacttgttgtggtgtttcatcattgaaagggggaattcctgttagaaattcaaacaagcaaactccaagtgcccaccagtctaccgcaggaccatgggccctgcctagtaacagctcaggtgcaaggtagtctggggttcctagaattcgcccatcatcaacgggggccacccctcttctcacactcttcggagttcggtatggagttcccgacttgatctgatttggggtctgctgatgtggcatacaggatcttcttttttgagtaggggttatagccatgggatatgaaccactgtaggcacacgaaatatccattgcatctaaagaagtcatgttcattctggatggttctgagttattggatgcattaatatgactgttaaaacttcgaaaagcaacagcatttcttttagaggctaacgttttcagcacctccaaaggaggacctaacattttttggttactctcttgtacagcagggttctcgacaccttttggtgaggtcttttcttggcaatctggtgttacaataagtggatcttcaatatttgattcttcaaaagaggattctttgatgcttctatctgaatctaagggctgactttctaatggactttccattatagaaattccaggaaaagatgaatcagagttcatagaaatatttttagaagctctatcatcatcagaacatagaaaactagaacttaagtagtccctcttactattcttttcacagtcttcatcgagttcacacataaggttttttgctatcattggtataggtaatttttctggtgtttgttgtttatcagtaaaagaattgacaatgttctccttattagcacagtcattttgttgacttttgtgcactgatagcttaaggtcctgcacttcaactgttaagcctgtattttgatttgtataacaatttgtcatttcgttatgcttatactctacacaagtttttttattctgtataatttttttacaaggactggagtcaaccaactcaaaatttctttttaaacttcttttcccaaggtgctcttcagatatcccaccagaatccacagcccactgatttgactgatggaaacctaactgacttgtgtcagtgtccatatttatattatttacatccagttctactgcttcccaagaaacttccccagagaagcattttttagcaaggtttacacaagagcgtccagtggtgggaagggcactgctgttatgaatgggagaaagagctaactccagatcctttttattgaaacctttcgtctcaatggcatttgcagattttgcgcataacttttcaactgcattccaactcatcattgttgggcccaatgcttcatcactttcctggcaatctttttcccatttgggactgctgtggcattctgattccacactggatatgaaggtgtgggattgactactggcactggatgtggccagccttttcctagactggagtaaattagaagttagacacttcacaggcattcctgggttggaggcaactgtttcaagacatgattttagtaatttgctagaataaggcgtagtgtccttttgatctacagacatagggcatacgagtccttgagaaagctgtgatgtttcagacagacaggctgaaaggatgtttgcagggtcttgatttttttctgcaattggtgtgttaaatcccaacgagctgataagcgataacacttgtcctggggttcttgaataatcttgtctaggttttgccattgatggtgttgtaaggatatccatcatattaatatctctattcaaagtaacttttgaaaggccaaaatccgtcagtttaatatgaccctcattagaaataagcatattgtccggtttcaagtccctgtggatgattccatgtctgtgaaggtagtctagagccagtgctacttcagaaatatatttcacagccatctcttcatcaaaataaccatatatatgtaggagagacttgacatctcccccaataagatattccattaccaagtagacattgtttgcagactgcagtgaataatacaaatggacaatgaatgggcttttgcttagtgccagtgcatctctctcagcttggacctgatgagtcatatttttgttgatcatgtctgcttttttaacaacctttactgcatacaatttgccgcctttctgccccagatacactttcccgaaggcgccccggctaatgggcttcactatgctgaattcctcaatggagggcggttttggcactgcgatcctattcacgccctcctcagtcgccgcgcctcctccaggctccttcttgcttcccgcggtgggatccatcgctggacagcatacagcggccccgcagacactgcccctccgcgagcagccactcccgccaactgggttcaaagt

SEQ ID NO: 15970 - RNA, 3695 nt, Homo sapiens
  source 1..3695: mol_type = other RNA
gctgggattacaggcatgagccatcgcacccgtcctccagtaccattttaaacaaatacatattgtggactacgcaccaatagaaattaaggtggcaaaaccgtatcattagtaaagtaagtgaaagccttagtctttttgtttattccttattccccaaaggagttactaagtgaaggaattttccagctgcctttatttttttgagacggagtcttgttctgttgcccaggctggagtgcagtggcacgatcttggctcaccacaacctcctcctcctgggttccagcgattctcctgcctcagcctccagagtagctgggactacaggcgcccaccaacatgcccggctaatttgtgtatttacagtagagatggggtttcattatgttggccaggatggtcttgaactcctgacctcaagatcagcctgcctcggcctcccacagtgctgggattacatgcgtgagccactgcgcccggccttccagctgcatttctgaggtcacaagtatggccttaaatgattgccctcaagaacacagcttttgaaggtaatcatatgcaagtaaattacaatcaaatggaactgtatgattattttattattttaatgctaaactgaacagtgaactgaaatcagaggagaaagaaaatcaagctagtggctcactctcaatagtgtcctctaattttattgatgcttcagttttcataaagtgcaataaacaaaataaataaatgaaaaaagctttgaagatttatatacagttttgaggttaagataaattactgactatattcctttcagccttttaactctgtgaaagctgtaacgtacattaaaagcacattgaactaggttaaataatgatctttcccccttagatcaatctagtattaaggagtatataattatgcaagttcattctataacacaaggctagactaaaaggaaaatttttgtgctacagactaaatccagatacagtcaggtgctgagcagtattcctggcttcaaaataggaggtatctgtttcatcatctggctgggggatgaaaggcatagtctgatgctgcagattttcccagtccacatcactgaagagaggatgacgttttagctctttcattccagctctctttgtatcatcaatggttaaaagtatttctactgcactttgagcattatcagataacttttcttcaccttctggccaagggatatctcttttcagaatattctggaatacttgttgtggtgtttcatcattgaaagggggaattcctgttagaaattcaaacaagcaaactccaagtgcccaccagtctaccgcaggaccggaagtcagaaatccatgggccctgcctagtaacagctcaggtgcaaggtagtctggggttcctagaattcgcccatcatcaacgggggccacccctcttctcacactcttcggagttcggtatggagttcccgacttgatctgatttggggtctgatgtggcatacaggatcttcttttttgagtaggggttatagccatgggatatgaaccactgtaggcacacgaaatatccattgcatctaaagaagtcatgttcattctggatggttctgagttattggatgcattaatatgactgttaaaacttcgaaaagcaacagcatttcttttagaggctaacgttttcagcacctccaaaggaggacctaacattttttggttactctcttgtacagcagggttctcgacaccttttggtgaggtcttttcttggcaatctggtgttacaataagtggatcttcaatatttgattcttcaaaagaggattctttgatgcttctatctgaatctaagggctgactttctaatggactttccattatagaaattccaggaaaagatgaatcagagttcatagaaatatttttagaagctctatcatcatcagaacatagaaaactagaacttaagtagtccctcttactattcttttcacagtcttcatcgagttcacacataaggttttttgctatcattggtataggtaatttttctggtgtttgttgtttatcagtaaaagaattgacaatgttctccttattagcacagtcattttgttgacttttgtgcactgatagcttaaggtcctgcacttcaactgttaagcctgtattttgatttgtataacaatttgtcatttcgttatgcttatactctacacaagtttttttattctgtataatttttttacaaggactggagtcaaccaactcaaaatttctttttaaacttcttttcccaaggtgctcttcagatatcccaccagaatccacagcccactgatttgactgatggaaacctaactgacttgtgtcagtgtccatatttatattatttacatccagttctactgcttcccaagaaacttccccagagaagcattttttagcaaggtttacacaagagcgtccagtggtgggaagggcactgctgttatgaatgggagaaagagctaactccagatcctttttattgaaacctttcgtctcaatggcatttgcagattttgcgcataacttttcaactgcattccaactcatcattgttgggcccaatgcttcatcactttcctggcaatctttttcccatttgggactgctgtggcattctgattccacactggatatgaaggtgtgggattgactactggcactggatgtggccagccttttcctagactggagtaaattagaagttagacacttcacaggcattcctgggttggaggcaactgtttcaagacatgattttagtaatttgctagaataaggcgtagtgtccttttgatctacagacatagggcatacgagtccttgagaaagctgtgatgtttcagacagacaggctgaaaggatgtttgcagggtcttgatttttttctgcaattggtgtgttaaatcccaacgagctgataagcgataacacttgtcctggggttcttgaataatcttgtctaggttttgccattgatggtgttgtaaggatatccatcatattaatatctctattcaaagtaacttttgaaaggccaaaatccgtcagtttaatatgaccctcattagaaataagcatattgtccggtttcaagtccctgtggatgattccatgtctgtgaaggtagtctagagccagtgctacttcagaaatatatttcacagccatctcttcatcaaaataaccatatatatgtaggagagacttgacatctcccccaataagatattccattaccaagtagacattgtttgcagactgcagtgaataatacaaatggacaatgaatgggcttttgcttagtgccagtgcatctctctcagcttggacctgatgagtcatatttttgttgatcatgtctgcttttttaacaacctttactgcatacaatttgccgcctttctgccccagatacactttcccgaaggcgccccggctaatgggcttcactatgctgaattcctcaatggagggcggttttggcactgcgatcctattcacgccctcctcagtcgccgcgcctcctccaggctccttcttgcttcccgcggtgggatccatcgctggacagcatacagcggccccgcagacactgcccctccgcgagcagccactcccgccaactgggttcaaagt

SEQ ID NO: 15971 - RNA, 2728 nt, Homo sapiens
  source 1..2728: mol_type = other RNA
gctgggattacaggcatgagccatcgcacccgtcctccagtaccattttaaacaaatacatattgtggactacgcaccaatagaaattaaggtggcaaaaccgtatcattagtaaagtaagtgaaagccttagtctttttgtttattccttattccccaaaggagttactaagtgaaggaattttccagctgcctttatttttttgagacggagtcttgttctgttgcccaggctggagtgcagtggcacgatcttggctcaccacaacctcctcctcctgggttccagcgattctcctgcctcagcctccagagtagctgggactacaggcgcccaccaacatgcccggctaatttgtgtatttacagtagagatggggtttcattatgttggccaggatggtcttgaactcctgacctcaagatcagcctgcctcggcctcccacagtgctgggattacatgcgtgagccactgcgcccggccttccagctgcatttctgaggtcacaagtatggccttaaatgattgccctcaagaacacagcttttgaaggtaatcatatgcaagtaaattacaatcaaatggaactgtatgattattttattattttaatgctaaactgaacagtgaactgaaatcagaggagaaagaaaatcaagctagtggctcactctcaatagtgtcctctaattttattgatgcttcagttttcataaagtgcaataaacaaaataaataaatgaaaaaagctttgaagatttatatacagttttgaggttaagataaattactgactatattcctttcagccttttaactctgtgaaagctgtaacgtacattaaaagcacattgaactaggttaaataatgatctttcccccttagatcaatctagtattaaggagtatataattatgcaagttcattctataacacaaggctagactaaaaggaaaatttttgtgctacagactaaatccagatacagtcaggtgctgagcagtattcctggcttcaaaataggaggtatctgtttcatcatctggctgggggatgaaaggcatagtctgatgctgcagattttcccagtccacatcactgaagagaggatgacgttttagctctttcattccagctctctttgtatcatcaatggttaaaagtatttctactgcactttgagcattatcagataacttttcttcaccttctggccaagggatatctcttttcagaatattctggaatacttgttgtggtgtttcatcattgaaagggggaattcctgttagaaattcaaacaagcaaactccaagtgcccaccagtctaccgcaggaccggaagtcagaaatccatgggccctgcctagtaacagctcaggtgcaaggtagtctggggttcctagaattcgcccatcatcaacgggggccacccctcttctcacactcttcggagttcggtatggagttcccgacttgatctgatttggggtctgctgatgtggcatacaggatcttcttttttgagtaggggttatagccatgggatatgaaccactgtaggcacacgaaatatccattgcatctaaagaagtcatgttcattctggatggttctgagttattggatgcattaatatgactgttaaaacttcgaaaagcaacagcatttcttttagaggctaacgttttcagcacctccaaaggaggacctaacattttttggttactctcttgtacagcagggttctcgacaccttttggtgaggtcttttcttggcaatctggtgttacaataagtggatcttcaatatttgattcttcaaaagaggattctttgatgcttctatctgaatctaagggctgactttctaatggactttccattatagaaattccaggaaaagatgaatcagagttcatagaaatatttttagaagctctatcatcatcagaacatagaaaactagaacttaagtagtccctcttactattcttttcacagtcttcatcgagttcacacataaggttttttgctatcattggtataggtaatttttctggtgtttgttgtttatcagtaaaagaattgacaatgttctccttattagcacagtcattttgttgacttttgtgcactgatagcttaaggtcctgcacttcaactgttaagcctgtattttgatttgtataacaatttgtcatttcgttatgcttatactctacacaagtttttttattctgtataatttttttacaaggactggagtcaaccaactcaaaatttctttttaaacttcttttcccaaggtgctcttcagatatcccaccagaatccacagcccactgatttgactgatggaaacctaactgacttgtgtcagtgtccatatttatattatttacatccagttctactgcttcccaagaaacttccccagagaagcattttttagcaaggtttacacaagagcgtccagtggtgggaagggcactgctgttatgaatgggagaaagagctaactccagatcctttttattgaaacctttcgtctcaatggcatttgcagattttgcgcataacttttcaactgcattccaactcatcattgttgggcccaatgcttcatcactttcatgattttagtaatttgctagaataaggcgtagtgtccttttgatctacagacatagggcatacgagtccttgagaaagctgtgatgtt

SEQ ID NO: 15972 - RNA, 3818 nt, Homo sapiens
  source 1..3818: mol_type = other RNA
gctgggattacaggcatgagccatcgcacccgtcctccagtaccattttaaacaaatacatattgtggactacgcaccaatagaaattaaggtggcaaaaccgtatcattagtaaagtaagtgaaagccttagtctttttgtttattccttattccccaaaggagttactaagtgaaggaattttccagctgcctttatttttttgagacggagtcttgttctgttgcccaggctggagtgcagtggcacgatcttggctcaccacaacctcctcctcctgggttccagcgattctcctgcctcagcctccagagtagctgggactacaggcgcccaccaacatgcccggctaatttgtgtatttacagtagagatggggtttcattatgttggccaggatggtcttgaactcctgacctcaagatcagcctgcctcggcctcccacagtgctgggattacatgcgtgagccactgcgcccggccttccagctgcatttctgaggtcacaagtatggccttaaatgattgccctcaagaacacagcttttgaaggtaatcatatgcaagtaaattacaatcaaatggaactgtatgattattttattattttaatgctaaactgaacagtgaactgaaatcagaggagaaagaaaatcaagctagtggctcactctcaatagtgtcctctaattttattgatgcttcagttttcataaagtgcaataaacaaaataaataaatgaaaaaagctttgaagatttatatacagttttgaggttaagataaattactgactatattcctttcagccttttaactctgtgaaagctgtaacgtacattaaaagcacattgaactaggttaaataatgatctttcccccttagatcaatctagtattaaggagtatataattatgcaagttcattctataacacaaggctagactaaaaggaaaatttttgtgctacagactaaatccagatacagtcaggtgctgagcagtattcctggcttcaaaataggaggtatctgtttcatcatctggctgggggatgaaaggcatagtctgatgctgcagattttcccagtccacatcactgaagagaggatgacgttttagctctttcattccagctctctttgtatcatcaatggttaaaagtatttctactgcactttgagcattatcagataacttttcttcaccttctggccaagggatatctcttttcagaatattctggaatacttgttgtggtgtttcatcattgaaagggggaattcctgttagaaattcaaacaagcaaactccaagtgcccaccagtctaccgcaggaccggaagtcagaaatccatgggccctgcctagtaacagctcaggtgcaaggtagtctggggttcctagaattcgcccatcatcaacgggggccacccctcttctcacactcttcggagttcggtatggagttcccgacttgatctgatttggggtctgctgatgtggcatacaggatcttcttttttgagtaggggttatagccatgggatatgaaccactgtaggcacacgaaatatccattgcatctaaagaagtcatgttcattctggatggttctgagttattggatgcattaatatgactgttaaaacttcgaaaagcaacagcatttcttttagaggctaacgttttcagcacctccaaaggaggacctaacattttttggttactctcttgtacagcagggttctcgacaccttttggtgaggtcttttcttggcaatctggtgttacaataagtggatcttcaatatttgattcttcaaaagaggattctttgatgcttctatctgaatctaagggctgactttctaatggactttccattatagaaattccaggaaaagatgaatcagagttcatagaaatatttttagaagctctatcatcatcagaacatagaaaactagaacttaagtagtccctcttactattcttttcacagtcttcatcgagttcacacataaggttttttgctatcattggtataggtaatttttctggtgtttgttgtttatcagtaaaagaattgacaatgttctccttattagcacagtcattttgttgacttttgtgcactgatagcttaaggtcctgcacttcaactgttaagcctgtattttgatttgtataacaatttgtcatttcgttatgcttatactctacacaagtttttttattctgtataatttttttacaaggactggagtcaaccaactcaaaatttctttttaaacttcttttcccaaggtgctcttcagatatcccaccagaatccacagcccactgatttgactgatggaaacctaactgacttgtgtcagtgtccatatttatattatttacatccagttctactgcttcccaagaaacttccccagagaagcattttttagcaaggtttacacaagagcgtccagtggtgggaagggcactgctgttatgaatgggagaaagagctaactccagatcctttttattgaaacctttcgtctcaatggcatttgcagattttgcgcataacttttcaactgcattccaactcatcattgttgggcccaatgcttcatcactttcctggcaatctttttcccatttgggactgctgtggcattctgattccacactggatatgaaggtgtgggattgactactggcactggatgtggccagccttttcctagactggagtaaattagaagttagacacttcacaggcattcctgggttggaggcaactgtttcaagacatgattttagtaatttgctagaataaggcgtagtgtccttttgatctacagacatagggcatacgagtccttgagaaagctgtgatgtttcagacagacaggctgaaaggatgtttgcagggtcttgatttttttctgcaattggtgtgttaaatcccaacgagctgataagcgataacacttgtcctggggttcttgaataatcttgtctaggttttgccattgatggtgttgtaaggatatccatcatattaatatctctattcaaagtaacttttgaaaggccaaaatccgtcagtttaatatgaccctcattagaaataagcatattgtccggtttcaagtccctctactcccagacacttgggaggctaaggcagggggattgcttgagccccagaggtcgaggctgcagtgagccaaggtcaagtcactgcactgcacaacctggatgacaaagtgagaccctgtggatgattccatgtctgtgaaggtagtctagagccagtgctacttcagaaatatatttcacagccatctcttcatcaaaataaccatatatatgtaggagagacttgacatctcccccaataagatattccattaccaagtagacattgtttgcagactgcagtgaataatacaaatggacaatgaatgggcttttgcttagtgccagtgcatctctctcagcttggacctgatgagtcatatttttgttgatcatgtctgcttttttaacaacctttactgcatacaatttgccgcctttctgccccagatacactttcccgaaggcgccccggctaatgggcttcactatgctgaattcctcaatggagggcggttttggcactgcgatcctattcacgccctcctcagtcgccgcgcctcctccaggctccttcttgcttcccgcggtgggatccatcgctggacagcatacagcggccccgcagacactgcccctccgcgagcagccactcccgccaactgggttcaaagt

SEQ ID NO: 15973 - RNA, 3698 nt, Homo sapiens
  source 1..3698: mol_type = other RNA
gctgggattacaggcatgagccatcgcacccgtcctccagtaccattttaaacaaatacatattgtggactacgcaccaatagaaattaaggtggcaaaaccgtatcattagtaaagtaagtgaaagccttagtctttttgtttattccttattccccaaaggagttactaagtgaaggaattttccagctgcctttatttttttgagacggagtcttgttctgttgcccaggctggagtgcagtggcacgatcttggctcaccacaacctcctcctcctgggttccagcgattctcctgcctcagcctccagagtagctgggactacaggcgcccaccaacatgcccggctaatttgtgtatttacagtagagatggggtttcattatgttggccaggatggtcttgaactcctgacctcaagatcagcctgcctcggcctcccacagtgctgggattacatgcgtgagccactgcgcccggccttccagctgcatttctgaggtcacaagtatggccttaaatgattgccctcaagaacacagcttttgaaggtaatcatatgcaagtaaattacaatcaaatggaactgtatgattattttattattttaatgctaaactgaacagtgaactgaaatcagaggagaaagaaaatcaagctagtggctcactctcaatagtgtcctctaattttattgatgcttcagttttcataaagtgcaataaacaaaataaataaatgaaaaaagctttgaagatttatatacagttttgaggttaagataaattactgactatattcctttcagccttttaactctgtgaaagctgtaacgtacattaaaagcacattgaactaggttaaataatgatctttcccccttagatcaatctagtattaaggagtatataattatgcaagttcattctataacacaaggctagactaaaaggaaaatttttgtgctacagactaaatccagatacagtcaggtgctgagcagtattcctggcttcaaaataggaggtatctgtttcatcatctggctgggggatgaaaggcatagtctgatgctgcagattttcccagtccacatcactgaagagaggatgacgttttagctctttcattccagctctctttgtatcatcaatggttaaaagtatttctactgcactttgagcattatcagataacttttcttcaccttctggccaagggatatctcttttcagaatattctggaatacttgttgtggtgtttcatcattgaaagggggaattcctgttagaaattcaaacaagcaaactccaagtgcccaccagtctaccgcaggaccggaagtcagaaatccatgggccctgcctagtaacagctcaggtgcaaggtagtctggggttcctagaattcgcccatcatcaacgggggccacccctcttctcacactcttcggagttcggtatggagttcccgacttgatctgatttggggtctgctgatgtggcatacaggatcttcttttttgagtaggggttatagccatgggatatgaaccactgtaggcacacgaaatatccattgcatctaaagaagtcatgttcattctggatggttctgagttattggatgcattaatatgactgttaaaacttcgaaaagcaacagcatttcttttagaggctaacgttttcagcacctccaaaggaggacctaacattttttggttactctcttgtacagcagggttctcgacaccttttggtgaggtcttttcttggcaatctggtgttacaataagtggatcttcaatatttgattcttcaaaagaggattctttgatgcttctatctgaatctaagggctgactttctaatggactttccattatagaaattccaggaaaagatgaatcagagttcatagaaatatttttagaagctctatcatcatcagaacatagaaaactagaacttaagtagtccctcttactattcttttcacagtcttcatcgagttcacacataaggttttttgctatcattggtataggtaatttttctggtgtttgttgtttatcagtaaaagaattgacaatgttctccttattagcacagtcattttgttgacttttgtgcactgatagcttaaggtcctgcacttcaactgttaagcctgtattttgatttgtataacaatttgtcatttcgttatgcttatactctacacaagtttttttattctgtataatttttttacaaggactggagtcaaccaactcaaaatttctttttaaacttcttttcccaaggtgctcttcagatatcccaccagaatccacagcccactgatttgactgatggaaacctaactgacttgtgtcagtgtccatatttatattatttacatccagttctactgcttcccaagaaacttccccagagaagcattttttagcaaggtttacacaagagcgtccagtggtgggaagggcactgctgttatgaatgggagaaagagctaactccagatcctttttattgaaacctttcgtctcaatggcatttgcagattttgcgcataacttttcaactgcattccaactcatcattgttgggcccaatgcttcatcactttcctggcaatctttttcccatttgggactgctgtggcattctgattccacactggatatgaaggtgtgggattgactactggcactggatgtggccagccttttcctagactggagtaaattagaagttagacacttcacaggcattcctgggttggaggcaactgtttcaagacatgattttagtaatttgctagaataaggcgtagtgtccttttgatctacagacatagggcatacgagtccttgagaaagctgtgatgtttcagacagacaggctgaaaggatgtttgcagggtcttgatttttttctgcaattggtgtgttaaatcccaacgagctgataagcgataacacttgtcctggggttcttgaataatcttgtctaggttttgccattgatggtgttgtaaggatatccatcatattaatatctctattcaaagtaacttttgaaaggccaaaatccgtcagtttaatatgaccctcattagaaataagcatattgtccggtttcaagtccctgtggatgattccatgtctgtgaaggtagtctagagccagtgctacttcagaaatatatttcacagccatctcttcatcaaaataaccatatatatgtaggagagacttgacatctcccccaataagatattccattaccaagtagacattgtttgcagactgcagtgaataatacaaatggacaatgaatgggcttttgcttagtgccagtgcatctctctcagcttggacctgatgagtcatatttttgttgatcatgtctgcttttttaacaacctttactgcatacaatttgccgcctttctgccccagatacactttcccgaaggcgccccggctaatgggcttcactatgctgaattcctcaatggagggcggttttggcactgcgatcctattcacgccctcctcagtcgccgcgcctcctccaggctccttcttgcttcccgcggtgggatccatcgctggacagcatacagcggccccgcagacactgcccctccgcgagcagccactcccgccaactgggttcaaagt

SEQ ID NO: 15974 - RNA, 3541 nt, Homo sapiens
  source 1..3541: mol_type = other RNA
gctgggattacaggcatgagccatcgcacccgtcctccagtaccattttaaacaaatacatattgtggactacgcaccaatagaaattaaggtggcaaaaccgtatcattagtaaagtaagtgaaagccttagtctttttgtttattccttattccccaaaggagttactaagtgaaggaattttccagctgcctttatttttttgagacggagtcttgttctgttgcccaggctggagtgcagtggcacgatcttggctcaccacaacctcctcctcctgggttccagcgattctcctgcctcagcctccagagtagctgggactacaggcgcccaccaacatgcccggctaatttgtgtatttacagtagagatggggtttcattatgttggccaggatggtcttgaactcctgacctcaagatcagcctgcctcggcctcccacagtgctgggattacatgcgtgagccactgcgcccggccttccagctgcatttctgaggtcacaagtatggccttaaatgattgccctcaagaacacagcttttgaaggtaatcatatgcaagtaaattacaatcaaatggaactgtatgattattttattattttaatgctaaactgaacagtgaactgaaatcagaggagaaagaaaatcaagctagtggctcactctcaatagtgtcctctaattttattgatgcttcagttttcataaagtgcaataaacaaaataaataaatgaaaaaagctttgaagatttatatacagttttgaggttaagataaattactgactatattcctttcagccttttaactctgtgaaagctgtaacgtacattaaaagcacattgaactaggttaaataatgatctttcccccttagatcaatctagtattaaggagtatataattatgcaagttcattctataacacaaggctagactaaaaggaaaatttttgtgctacagactaaatccagatacagtcaggtgctgagcagtattcctggcttcaaaataggaggtatctgtttcatcatctggctgggggatgaaaggcatagtctgatgctgcagattttcccagtccacatcactgaagagaggatgacgttttagctctttcattccagctctctttgtatcatcaatggttaaaagtatttctactgcactttgagcattatcagataacttttcttcaccttctggccaagggatatctcttttcagaatattctggaatacttgttgtggtgtttcatcattgaaagggggaattcctgttagaaattcaaacaagcaaactccaagtgcccaccagtctaccgcaggacctgatgtggcatacaggatcttcttttttgagtaggggttatagccatgggatatgaaccactgtaggcacacgaaatatccattgcatctaaagaagtcatgttcattctggatggttctgagttattggatgcattaatatgactgttaaaacttcgaaaagcaacagcatttcttttagaggctaacgttttcagcacctccaaaggaggacctaacattttttggttactctcttgtacagcagggttctcgacaccttttggtgaggtcttttcttggcaatctggtgttacaataagtggatcttcaatatttgattcttcaaaagaggattctttgatgcttctatctgaatctaagggctgactttctaatggactttccattatagaaattccaggaaaagatgaatcagagttcatagaaatatttttagaagctctatcatcatcagaacatagaaaactagaacttaagtagtccctcttactattcttttcacagtcttcatcgagttcacacataaggttttttgctatcattggtataggtaatttttctggtgtttgttgtttatcagtaaaagaattgacaatgttctccttattagcacagtcattttgttgacttttgtgcactgatagcttaaggtcctgcacttcaactgttaagcctgtattttgatttgtataacaatttgtcatttcgttatgcttatactctacacaagtttttttattctgtataatttttttacaaggactggagtcaaccaactcaaaatttctttttaaacttcttttcccaaggtgctcttcagatatcccaccagaatccacagcccactgatttgactgatggaaacctaactgacttgtgtcagtgtccatatttatattatttacatccagttctactgcttcccaagaaacttccccagagaagcattttttagcaaggtttacacaagagcgtccagtggtgggaagggcactgctgttatgaatgggagaaagagctaactccagatcctttttattgaaacctttcgtctcaatggcatttgcagattttgcgcataacttttcaactgcattccaactcatcattgttgggcccaatgcttcatcactttcctggcaatctttttcccatttgggactgctgtggcattctgattccacactggatatgaaggtgtgggattgactactggcactggatgtggccagccttttcctagactggagtaaattagaagttagacacttcacaggcattcctgggttggaggcaactgtttcaagacatgattttagtaatttgctagaataaggcgtagtgtccttttgatctacagacatagggcatacgagtccttgagaaagctgtgatgtttcagacagacaggctgaaaggatgtttgcagggtcttgatttttttctgcaattggtgtgttaaatcccaacgagctgataagcgataacacttgtcctggggttcttgaataatcttgtctaggttttgccattgatggtgttgtaaggatatccatcatattaatatctctattcaaagtaacttttgaaaggccaaaatccgtcagtttaatatgaccctcattagaaataagcatattgtccggtttcaagtccctgtggatgattccatgtctgtgaaggtagtctagagccagtgctacttcagaaatatatttcacagccatctcttcatcaaaataaccatatatatgtaggagagacttgacatctcccccaataagatattccattaccaagtagacattgtttgcagactgcagtgaataatacaaatggacaatgaatgggcttttgcttagtgccagtgcatctctctcagcttggacctgatgagtcatatttttgttgatcatgtctgcttttttaacaacctttactgcatacaatttgccgcctttctgccccagatacactttcccgaaggcgccccggctaatgggcttcactatgctgaattcctcaatggagggcggttttggcactgcgatcctattcacgccctcctcagtcgccgcgcctcctccaggctccttcttgcttcccgcggtgggatccatcgctggacagcatacagcggccccgcagacactgcccctccgcgagcagccactcccgccaactgggttcaaagt

SEQ ID NO: 15975 - RNA, 6602 nt, Homo sapiens
  source 1..6602: mol_type = other RNA
gctgggattacaggcatgagccatcgcacctggccagtttttttttttttttttttttctaagtgcaatgggaagccactcaaagggctttaagcagggaagtgacattatctgattttcgttttataaagatccctgcggctgccgtcagtgattgtaggagggcaggagtggatgcaaggacagcagacattagtgcaggagttcaggtgaaagatgataatagcttgggcagagtggtagcagtggacatggagggaggtagacagatttaagatgtctcggagacagctgatggaatttgctgataactggaatgggagtgacaatgacaaataaaggaacctagaataagccccagaattttgcttaagcaactgagagttcagccatggcagatctgttaagcacaaaagttaaacacaaatacaaattcatactgcattggactcttttaagcagtgtcttatagaaaaaacattttatctagggaaaaatgcaacaacaaaaaccactgaaaacaaaagcctatgaataaaagcagacccgttttagactggatgcacaaaacaaaaacacacaggattcttgtggtggcgatgggagtaagtgaagacgtaacaggttgcaagttattttaaggactaagacccaatgttcagaaaccaaatcttgttcttccagtgtggatgcttagtcaaagactgtaaattgtcttcaagctgagagagaccatgaagagagaggagtggccacctaactaaccttcccagtttttgggagccaaacctagaccagaatgtaggtctaagtgactcccaatccagagctgtctccattaggccaggctctcaccccagctccaaaccaacttctaaaaacttgtccaagagtcctcctcttctttagaattggtaatcttggcaattaaattcagcgtagaaacactctcctgaacataatcagcatgctggttcttccttttctgttgccttgctcttcctaacagctcctcctttcgtctttgcaggctgcttctctgtcacaggaactcagggctcagtgctgtacttcatctccaaagtgtccctaaagcgcccatctgatcccatggctaactactccccaaattttctcctggactgaccttactgaatttagatttgtacatccaatacctgcttaacatatccactttgatgctcagtgggcacctcacacttgatctgtcaaacactgaatttctgtctctgttatgcacatacccaaactttccccaccatgtatttccccatctcaataaactgcaatagctcaagccaaaagcctaagattcagacctgaattctttcctttcctctctctcaaatgcaattcaacaattttcttaccttttattttttgttttggaatgaaggcacatataactgagctagtaataatgcttgattcataatacaccaccgatgttccatgcataactctcttattcatttgtccatgcatttattttgtttttgaatttttttaaaggggggcaaggtctacgttgcccaggttggaatatagtagctattcacaggtgaaatcatagcacactatagccttgaactggcctcaaggatcttcctatctcagactcccaagtagctgggactataagcacgcaccactacacccagctcatgtacttacttttaatgacaaatgaaccaccccaaaacccaccacctaacccagggactaaaacattaccagtgacttactcatagatttgctcctcctctacctctccagaggtaaccactatcttgaactttattactttttaaaagttttgtcacatatgtcaatgcctaaacagctgttcagttttagttgttcttgacttttataagaaaagtatcatgtcacatatagttttctcagaattgctttttcattctgagttattgtgctgcaagtagctggtattcattcattttgctgccatgtaataatcacccattctgtgaacacattacaccttcctaaaaatagacattttaatttattccagaacattcttatatgtgtgatctgggggacctgtgcaagcatttctcaagtatatactgaaaagtgaaattgctgacccatgggtatactttttttttttttttaaggtatgatcttactctgtcacccaaggtaagagtgcagtggcacaatcatgattcactgcagcctcaacctcctgggcttaagcaatccttccacctcagcttcccaagtagctgggaccacaggcatgcaccaccatgcccagctaattcaaaaaaatctttttgtgcagatgtggtctccctatgttgctcaagctggtcttgaactcttgggctcaagtgatcctcctaccttggcctcccaaagccaagaggcatgagccactgggcctggcccaacttttctagtgaatggtttttcacagtggatataccaattgatacccccatcagcaatatgtgagtgatcctaatgactaaaaccctctccaaaacttgactttgtgtttcttcattttcaccaatcgaatgaatttgaacatgtcattgtcatcttgatttacgttttcctgattgagagatgaaaacctcttaatgtttattggcccacatgcacttctaattgtgtggaaggcctggttcagtcttttgcctgtttttctgtgacactgtccttttttgttggtttgtagaatttctgcatacattcttgatactaagctattactagttataaatgttgcagatattgcctcacagtttgtagtttagctttagttttttttttagagacaaggtctccctatgttgcccaagttggacttgaacccctgggctcaagcaatcctcccacctcatcctcccaagttcatggacacagtgtgtgtgtgtgtgtgtgtgtgtgtgtgtgtgtaaatggagtttccctatttttcccaggcccgtctcaaactcctgggctcaagcagctcaagtaatccttctgcctctgcctcccaaagtgctgggattacaggcatgagccacaatgcctaactactgatgcacgatttctaaattaagaatttataatataccataacttatattcttttatggttatcttttatggtttttttttttcctgcttccagtttaagaagttcttcctaaagggagtaggatcaggaagataatcacattttctaaatatgtttcaatcacattttaatctataattccacatatagtttctacatcaagtcgtcatcctgttgcattaattttaaagagcatgcttctagtgtataaggttgaaaagcattcttccccttatagattactaaagatttattattaatgggtatactgattttctttagtcttactttttatttatcctttttaagtcatcaacaaactttttctgagtatttgattacctttctttcaaaccgtacagtatctcctggatttgtttctctttttatttaggtactttctccaaaagtgattttagtttgtacggaaaatcttctgaagctttgatggtacatattcttattaatgccctcacattagaataactattttcagaacataaaattgtaggttcaaagtttttttcaggttcaatttcacattcttgagctaggcatggtactgatggttttcaccataacatacaccaatgtccttttgtctgtgggctcccatccagcctggtggctgaagtcatctacaggtaagattgaccaaacctctgaacaggactgaaaaaaatgttatcttcagaaaaccagccctcttgtacactgctgctgtgaatacaaattgattaacttttctggatggcaatctagcaatgcagatcaaacatttaaaaatacatatatatctcgacacaattttatctccaggcatccacatgaaagaactccacaatgttcagaagtgtacagataaggatactcgtcacagcattataatatgaaaaataaactgaaaaccacctcatctccaaacacaattaaattatgttaaaattctataaacagggattaggatgtgtaggtttacccaagggaaaatatatttaatgtttaggtttaaaaagcaaaaaaaaagcctactttttgtttcaaaaatatgcatatgtaagtagaaaatatctgaaagctgaaaggctactatccaaaaatattaacagcagctttctctaaacagaaactaaagcagtttctcttttctttttgcttttctatacttattacatgtctaccacaaacctctttgttataatttctccagttgagtcagttttacaatttggaatgcagagatcaagtggttctataatcagcatatacttcgcacgtaccattcattcaatccacacccctttaaacccctttgacacacgtcaaactcatttacatctatgtccctccaatgacaatatagtggtcaacacatataaaacatgaatacactatatcaagacactcaggaatacatctctgggataaaatctgactgccttctattatattttaatgaataaccaaaataaagggattctttcagttacagagagcagaataattaaaatagtaactttcaaactttgtagcagcagaagtatttcttcaaataaaatcttttttgaaacccaatatagaaaacagataaaaataaagccattctagaggtgggggccttggaaagtgagtactatccactcagacttctttcttgcctctcacaaggaaggaagctactgtgtagtttgaaaattactatttaatacattctgctaaccctaaatgccatgtcagagctagaagagaaaatgtacacacattcaatctaacatttatttatttcaggttttttttttttttggcaactataaattacattcactagtacacctggaattcttcatagtgtgttcaactaaagaataagcaaacacagcatagatcagtttaaaagaaatcatggtacttcttagagcaatttgcaaaaggggaaaaaagtcttaggctcactccttggaaataaatatcaagtaaccataaaaatattcagccatttttcagttattcggggagttcaggcatggtcccacgcagagcatcagagttcctctttgaaataacccagctttgccaatgacatctcttttctcaactgcataacctcccaaaacatctgatcaacatcctgctgtttcacgagtccctgctgaatgtatcgaatgtatgtaaaaaagttacatacagaagtgatcctgtatctgcaaaaaggagaaatataataatagttgcttgagtcccctaatttaattctgtgtttacaggacttactctggccagtgagagcacattttctcactttttgagaatgttaaacatggaaagatatcttcctggtagattttgtctaagaaaggacacgtcctgtccattgtgggctcatccttccacaatcggaattcattatacaaggataagtcagcctctttgcagtcttttacaattggctgtatcacactgaggtcctgatgactgccactcatagcactgcttgtgcttttatttcttgtatgcccctttttaaaaggtgtctttccacctggcaaaggctcctgcgtaggtgatgttggagaactggacaatacaagtgtcttcaatgcagctacttcagcttgaagtacatcaatttttccttgtgcttcttttagctgtttttctgctgttgcctgcttgatatttgcttctctcaccattttatgagcttcctcaaatagactagctgtgagttcttccaattcctgtccaagttgatctcgcacttttgaaagcctctcacattcttcatcttttaacttcagttccctctgagcttttgcgagttcttcttttaatcgttcatagcccttttctctaacttccaaaacagatgggcttcgtaaacgagacagactatcagtactcaacccaaaaatatcatcactgccatcgcaagcctctgttatagtagcaccctgtaaaaactctctctctgcattatagttgtcctttcttgtagttaatttagttaatccagctgtgactccagaggtagagcaaggggctgggtctgtaacatgaaagctgatactagatatttccgcacaatttaaacgtctgggggatgaatacacgggttgtgtaggaagttcagaaacatctaatgcatttgcctggataggtacagaggataaagctgaagggtgtggccggtagatgacacttggtgaggtagtctgctcttgagttcctgattcatacacaccaagaaggtccggagaagtaggtgaagcaaggtttacttcatggaagccttccaagggatcattagccatagcaaaagcctcatcataagataacctgagactccgcggccatatacaccttacgacgtgtgtgtgtgtggcgggagatgggaggggaggaatcctgtagaacccagatcccatcattccagcaactgccagagcgttcgagaatgtcatgtctgtacctgtcttct

SEQ ID NO: 15976 - RNA, 6820 nt, Homo sapiens
  source 1..6820: mol_type = other RNA
gctgggattacaggcatgagccatcgcacctggccagtttttttttttttttttttttctaagtgcaatgggaagccactcaaagggctttaagcagggaagtgacattatctgattttcgttttataaagatccctgcggctgccgtcagtgattgtaggagggcaggagtggatgcaaggacagcagacattagtgcaggagttcaggtgaaagatgataatagcttgggcagagtggtagcagtggacatggagggaggtagacagatttaagatgtctcggagacagctgatggaatttgctgataactggaatgggagtgacaatgacaaataaaggaacctagaataagccccagaattttgcttaagcaactgagagttcagccatggcagatctgttaagcacaaaagttaaacacaaatacaaattcatactgcattggactcttttaagcagtgtcttatagaaaaaacattttatctagggaaaaatgcaacaacaaaaaccactgaaaacaaaagcctatgaataaaagcagacccgttttagactggatgcacaaaacaaaaacacacaggattcttgtggtggcgatgggagtaagtgaagacgtaacaggttgcaagttattttaaggactaagacccaatgttcagaaaccaaatcttgttcttccagtgtggatgcttagtcaaagactgtaaattgtcttcaagctgagagagaccatgaagagagaggagtggccacctaactaaccttcccagtttttgggagccaaacctagaccagaatgtaggtctaagtgactcccaatccagagctgtctccattaggccaggctctcaccccagctccaaaccaacttctaaaaacttgtccaagagtcctcctcttctttagaattggtaatcttggcaattaaattcagcgtagaaacactctcctgaacataatcagcatgctggttcttccttttctgttgccttgctcttcctaacagctcctcctttcgtctttgcaggctgcttctctgtcacaggaactcagggctcagtgctgtacttcatctccaaagtgtccctaaagcgcccatctgatcccatggctaactactccccaaattttctcctggactgaccttactgaatttagatttgtacatccaatacctgcttaacatatccactttgatgctcagtgggcacctcacacttgatctgtcaaacactgaatttctgtctctgttatgcacatacccaaactttccccaccatgtatttccccatctcaataaactgcaatagctcaagccaaaagcctaagattcagacctgaattctttcctttcctctctctcaaatgcaattcaacaattttcttaccttttattttttgttttggaatgaaggcacatataactgagctagtaataatgcttgattcataatacaccaccgatgttccatgcataactctcttattcatttgtccatgcatttattttgtttttgaatttttttaaaggggggcaaggtctacgttgcccaggttggaatatagtagctattcacaggtgaaatcatagcacactatagccttgaactggcctcaaggatcttcctatctcagactcccaagtagctgggactataagcacgcaccactacacccagctcatgtacttacttttaatgacaaatgaaccaccccaaaacccaccacctaacccagggactaaaacattaccagtgacttactcatagatttgctcctcctctacctctccagaggtaaccactatcttgaactttattactttttaaaagttttgtcacatatgtcaatgcctaaacagctgttcagttttagttgttcttgacttttataagaaaagtatcatgtcacatatagttttctcagaattgctttttcattctgagttattgtgctgcaagtagctggtattcattcattttgctgccatgtaataatcacccattctgtgaacacattacaccttcctaaaaatagacattttaatttattccagaacattcttatatgtgtgatctgggggacctgtgcaagcatttctcaagtatatactgaaaagtgaaattgctgacccatgggtatactttttttttttttttaaggtatgatcttactctgtcacccaaggtaagagtgcagtggcacaatcatgattcactgcagcctcaacctcctgggcttaagcaatccttccacctcagcttcccaagtagctgggaccacaggcatgcaccaccatgcccagctaattcaaaaaaatctttttgtgcagatgtggtctccctatgttgctcaagctggtcttgaactcttgggctcaagtgatcctcctaccttggcctcccaaagccaagaggcatgagccactgggcctggcccaacttttctagtgaatggtttttcacagtggatataccaattgatacccccatcagcaatatgtgagtgatcctaatgactaaaaccctctccaaaacttgactttgtgtttcttcattttcaccaatcgaatgaatttgaacatgtcattgtcatcttgatttacgttttcctgattgagagatgaaaacctcttaatgtttattggcccacatgcacttctaattgtgtggaaggcctggttcagtcttttgcctgtttttctgtgacactgtccttttttgttggtttgtagaatttctgcatacattcttgatactaagctattactagttataaatgttgcagatattgcctcacagtttgtagtttagctttagttttttttttagagacaaggtctccctatgttgcccaagttggacttgaacccctgggctcaagcaatcctcccacctcatcctcccaagttcatggacacagtgtgtgtgtgtgtgtgtgtgtgtgtgtgtgtgtaaatggagtttccctatttttcccaggcccgtctcaaactcctgggctcaagcagctcaagtaatccttctgcctctgcctcccaaagtgctgggattacaggcatgagccacaatgcctaactactgatgcacgatttctaaattaagaatttataatataccataacttatattcttttatggttatcttttatggtttttttttttcctgcttccagtttaagaagttcttcctaaagggagtaggatcaggaagataatcacattttctaaatatgtttcaatcacattttaatctataattccacatatagtttctacatcaagtcgtcatcctgttgcattaattttaaagagcatgcttctagtgtataaggttgaaaagcattcttccccttatagattactaaagatttattattaatgggtatactgattttctttagtcttactttttatttatcctttttaagtcatcaacaaactttttctgagtatttgattacctttctttcaaaccgtacagtatctcctggatttgtttctctttttatttaggtactttctccaaaagtgattttagtttgtacggaaaatcttctgaagctttgatggtacatattcttattaatgccctcacattagaataactattttcagaacataaaattgtaggttcaaagtttttttcaggttcaatttcacattcttgagctaggcatggtactgatggttttcaccataacatacaccaatgtccttttgtctgtgggctcccatccagcctggtggctgaagtcatctacaggtaagattgaccaaacctctgaacaggactgaaaaaaatgttatcttcagaaaaccagccctcttgtacactgctgctgtgaatacaaattgattaacttttctggatggcaatctagcaatgcagatcaaacatttaaaaatacatatatatctcgacacaattttatctccaggcatccacatgaaagaactccacaatgttcagaagtgtacagataaggatactcgtcacagcattataatatgaaaaataaactgaaaaccacctcatctccaaacacaattaaattatgttaaaattctataaacagggattaggatgtgtaggtttacccaagggaaaatatatttaatgtttaggtttaaaaagcaaaaaaaaagcctactttttgtttcaaaaatatgcatatgtaagtagaaaatatctgaaagctgaaaggctactatccaaaaatattaacagcagctttctctaaacagaaactaaagcagtttctcttttctttttgcttttctatacttattacatgtctaccacaaacctctttgttataatttctccagttgagtcagttttacaatttggaatgcagagatcaagtggttctataatcagcatatacttcgcacgtaccattcattcaatccacacccctttaaacccctttgacacacgtcaaactcatttacatctatgtccctccaatgacaatatagtggtcaacacatataaaacatgaatacactatatcaagacactcaggaatacatctctgggataaaatctgactgccttctattatattttaatgaataaccaaaataaagggattctttcagttacagagagcagaataattaaaatagtaactttcaaactttgtagcagcagaagtatttcttcaaataaaatcttttttgaaacccaatatagaaaacagataaaaataaagccattctagaggtgggggccttggaaagtgagtactatccactcagacttctttcttgcctctcacaaggaaggaagctactgtgtagtttgaaaattactatttaatacattctgctaaccctaaatgccatgtcagagctagaagagaaaatgtacacacattcaatctaacatttatttatttcaggttttttttttttttggcaactataaattacattcactagtacacctggaattcttcatagtgtgttcaactaaagaataagcaaacacagcatagatcagtttaaaagaaatcatggtacttcttagagcaatttgcaaaaggggaaaaaagtcttaggctcactccttggaaataaatatcaagtaaccataaaaatattcagccatttttcagttattcggggagttcaggcatggtcccacgcagagcatcagagttcctctttgaaataacccagctttgccaatgacatctcttttctcaactgcataacctcccaaaacatctgatcaacatcctgctgtttcacgagtccctgctgaatgtatcgaatgtatgtaaaaaagttacatacagaagtgatcctgtatctgcaaaaaggagaaatataataatagttgcttgagtcccctaatttaattctgtgtttacaggacttactctggccagtgagagcacattttctctttgcagtcttttacaattggctgtatcacactgaggtcctgatgactgccactcatagcactgcttgtgcttttatttcttgtatgcccctttttaaaaggtgtctttccacctggcaaaggctcctgcgtaggtgatgttggagaactggacaatacaagtgtcttcaatgcagctacttcagcttgaagtacatcaatttttccttgtgcttcttttagctgtttttctgctgttgcctgcttgatatttgcttctctcaccattttatgagcttcctcaaatagactagctgtgagttcttccaattcctgtccaagttgatctcgcacttttgaaagcctctcacattcttcatcttttaacttcagttccctctgagcttttgcgagttcttcttttaatcgttcatagcccttttctctaacttccaaaacagatgggcttcgtaaacgagacagactatcagtactcaacccaaaaatatcatcactgccatcgcaagcctctgttatagtagcaccctgtaaaaactctctctctgcattatagttgtcctttcttgtagttaatttagttaatccagctgtgactccagaggtagagcaaggggctgggtctgtaacatgaaagctgatactagatatttccgcacaatttaaacgtctgggggatgaatacacgggttgtgtaggaagttcagaaacatctaatgcatttgcctggataggtacagaggataaagctgaagggtgtggccggtagatgacacttggtgaggtagtctgctcttgagttcctgattcatacacaccaagaaggtccggagaagtaggtgaagcaaggtttacttcatggaagccttccaagggatcattagccatagcaaaagcctcatcataagataaccctttcatcttttttaatcccataacaaccggcaactcttcacatgctgcgacttccacccagcatcatcacttctggagccagtaagctcgcgcttcctgggcggtcggggcgagttgtcaacgctgggagggcagagccatgcaatcccacccgtgcagttcgtctcaactcccccgaacacaagtctggcggcacggagctgcctacttgggcgcgactccgggcgcctgcccggaatttcccaccaggtttcaccgaaacctcccgagggtgacctctacgcctcagcacggtgcctcgcgcgtagtttcctaagactgggacacgaaaccaccccaggtccacagccctgccgcgcggcgtccggtgttgtgagctgcttccgacttgttcgggaactctctcttcatcctcttcgcgaccgcggccctccgctcccggccgcgcccgcccgccgccaggtaacccgctggactcgggctccct

SEQ ID NO: 15977 - RNA, 6503 nt, Homo sapiens
  source 1..6503: mol_type = other RNA
gctgggattacaggcatgagccatcgcacctggccagtttttttttttttttttttttctaagtgcaatgggaagccactcaaagggctttaagcagggaagtgacattatctgattttcgttttataaagatccctgcggctgccgtcagtgattgtaggagggcaggagtggatgcaaggacagcagacattagtgcaggagttcaggtgaaagatgataatagcttgggcagagtggtagcagtggacatggagggaggtagacagatttaagatgtctcggagacagctgatggaatttgctgataactggaatgggagtgacaatgacaaataaaggaacctagaataagccccagaattttgcttaagcaactgagagttcagccatggcagatctgttaagcacaaaagttaaacacaaatacaaattcatactgcattggactcttttaagcagtgtcttatagaaaaaacattttatctagggaaaaatgcaacaacaaaaaccactgaaaacaaaagcctatgaataaaagcagacccgttttagactggatgcacaaaacaaaaacacacaggattcttgtggtggcgatgggagtaagtgaagacgtaacaggttgcaagttattttaaggactaagacccaatgttcagaaaccaaatcttgttcttccagtgtggatgcttagtcaaagactgtaaattgtcttcaagctgagagagaccatgaagagagaggagtggccacctaactaaccttcccagtttttgggagccaaacctagaccagaatgtaggtctaagtgactcccaatccagagctgtctccattaggccaggctctcaccccagctccaaaccaacttctaaaaacttgtccaagagtcctcctcttctttagaattggtaatcttggcaattaaattcagcgtagaaacactctcctgaacataatcagcatgctggttcttccttttctgttgccttgctcttcctaacagctcctcctttcgtctttgcaggctgcttctctgtcacaggaactcagggctcagtgctgtacttcatctccaaagtgtccctaaagcgcccatctgatcccatggctaactactccccaaattttctcctggactgaccttactgaatttagatttgtacatccaatacctgcttaacatatccactttgatgctcagtgggcacctcacacttgatctgtcaaacactgaatttctgtctctgttatgcacatacccaaactttccccaccatgtatttccccatctcaataaactgcaatagctcaagccaaaagcctaagattcagacctgaattctttcctttcctctctctcaaatgcaattcaacaattttcttaccttttattttttgttttggaatgaaggcacatataactgagctagtaataatgcttgattcataatacaccaccgatgttccatgcataactctcttattcatttgtccatgcatttattttgtttttgaatttttttaaaggggggcaaggtctacgttgcccaggttggaatatagtagctattcacaggtgaaatcatagcacactatagccttgaactggcctcaaggatcttcctatctcagactcccaagtagctgggactataagcacgcaccactacacccagctcatgtacttacttttaatgacaaatgaaccaccccaaaacccaccacctaacccagggactaaaacattaccagtgacttactcatagatttgctcctcctctacctctccagaggtaaccactatcttgaactttattactttttaaaagttttgtcacatatgtcaatgcctaaacagctgttcagttttagttgttcttgacttttataagaaaagtatcatgtcacatatagttttctcagaattgctttttcattctgagttattgtgctgcaagtagctggtattcattcattttgctgccatgtaataatcacccattctgtgaacacattacaccttcctaaaaatagacattttaatttattccagaacattcttatatgtgtgatctgggggacctgtgcaagcatttctcaagtatatactgaaaagtgaaattgctgacccatgggtatactttttttttttttttaaggtatgatcttactctgtcacccaaggtaagagtgcagtggcacaatcatgattcactgcagcctcaacctcctgggcttaagcaatccttccacctcagcttcccaagtagctgggaccacaggcatgcaccaccatgcccagctaattcaaaaaaatctttttgtgcagatgtggtctccctatgttgctcaagctggtcttgaactcttgggctcaagtgatcctcctaccttggcctcccaaagccaagaggcatgagccactgggcctggcccaacttttctagtgaatggtttttcacagtggatataccaattgatacccccatcagcaatatgtgagtgatcctaatgactaaaaccctctccaaaacttgactttgtgtttcttcattttcaccaatcgaatgaatttgaacatgtcattgtcatcttgatttacgttttcctgattgagagatgaaaacctcttaatgtttattggcccacatgcacttctaattgtgtggaaggcctggttcagtcttttgcctgtttttctgtgacactgtccttttttgttggtttgtagaatttctgcatacattcttgatactaagctattactagttataaatgttgcagatattgcctcacagtttgtagtttagctttagttttttttttagagacaaggtctccctatgttgcccaagttggacttgaacccctgggctcaagcaatcctcccacctcatcctcccaagttcatggacacagtgtgtgtgtgtgtgtgtgtgtgtgtgtgtgtgtaaatggagtttccctatttttcccaggcccgtctcaaactcctgggctcaagcagctcaagtaatccttctgcctctgcctcccaaagtgctgggattacaggcatgagccacaatgcctaactactgatgcacgatttctaaattaagaatttataatataccataacttatattcttttatggttatcttttatggtttttttttttcctgcttccagtttaagaagttcttcctaaagggagtaggatcaggaagataatcacattttctaaatatgtttcaatcacattttaatctataattccacatatagtttctacatcaagtcgtcatcctgttgcattaattttaaagagcatgcttctagtgtataaggttgaaaagcattcttccccttatagattactaaagatttattattaatgggtatactgattttctttagtcttactttttatttatcctttttaagtcatcaacaaactttttctgagtatttgattacctttctttcaaaccgtacagtatctcctggatttgtttctctttttatttaggtactttctccaaaagtgattttagtttgtacggaaaatcttctgaagctttgatggtacatattcttattaatgccctcacattagaataactattttcagaacataaaattgtaggttcaaagtttttttcaggttcaatttcacattcttgagctaggcatggtactgatggttttcaccataacatacaccaatgtccttttgtctgtgggctcccatccagcctggtggctgaagtcatctacaggtaagattgaccaaacctctgaacaggactgaaaaaaatgttatcttcagaaaaccagccctcttgtacactgctgctgtgaatacaaattgattaacttttctggatggcaatctagcaatgcagatcaaacatttaaaaatacatatatatctcgacacaattttatctccaggcatccacatgaaagaactccacaatgttcagaagtgtacagataaggatactcgtcacagcattataatatgaaaaataaactgaaaaccacctcatctccaaacacaattaaattatgttaaaattctataaacagggattaggatgtgtaggtttacccaagggaaaatatatttaatgtttaggtttaaaaagcaaaaaaaaagcctactttttgtttcaaaaatatgcatatgtaagtagaaaatatctgaaagctgaaaggctactatccaaaaatattaacagcagctttctctaaacagaaactaaagcagtttctcttttctttttgcttttctatacttattacatgtctaccacaaacctctttgttataatttctccagttgagtcagttttacaatttggaatgcagagatcaagtggttctataatcagcatatacttcgcacgtaccattcattcaatccacacccctttaaacccctttgacacacgtcaaactcatttacatctatgtccctccaatgacaatatagtggtcaacacatataaaacatgaatacactatatcaagacactcaggaatacatctctgggataaaatctgactgccttctattatattttaatgaataaccaaaataaagggattctttcagttacagagagcagaataattaaaatagtaactttcaaactttgtagcagcagaagtatttcttcaaataaaatcttttttgaaacccaatatagaaaacagataaaaataaagccattctagaggtgggggccttggaaagtgagtactatccactcagacttctttcttgcctctcacaaggaaggaagctactgtgtagtttgaaaattactatttaatacattctgctaaccctaaatgccatgtcagagctagaagagaaaatgtacacacattcaatctaacatttatttatttcaggttttttttttttttggcaactataaattacattcactagtacacctggaattcttcatagtgtgttcaactaaagaataagcaaacacagcatagatcagtttaaaagaaatcatggtacttcttagagcaatttgcaaaaggggaaaaaagtcttaggctcactccttggaaataaatatcaagtaaccataaaaatattcagccatttttcagttattcggggagttcaggcatggtcccacgcagagcatcagagttcctctttgaaataacccagctttgccaatgacatctcttttctcaactgcataacctcccaaaacatctgatcaacatcctgctgtttcacgagtccctgctgaatgtatcgaatgtatgtaaaaaagttacatacagaagtgatcctgtatctgcaaaaaggagaaatataataatagttgcttgagtcccctaatttaattctgtgtttacaggacttactctggccagtgagagcacattttctctttgcagtcttttacaattggctgtatcacactgaggtcctgatgactgccactcatagcactgcttgtgcttttatttcttgtatgcccctttttaaaaggtgtctttccacctggcaaaggctcctgcgtaggtgatgttggagaactggacaatacaagtgtcttcaatgcagctacttcagcttgaagtacatcaatttttccttgtgcttcttttagctgtttttctgctgttgcctgcttgatatttgcttctctcaccattttatgagcttcctcaaatagactagctgtgagttcttccaattcctgtccaagttgatctcgcacttttgaaagcctctcacattcttcatcttttaacttcagttccctctgagcttttgcgagttcttcttttaatcgttcatagcccttttctctaacttccaaaacagatgggcttcgtaaacgagacagactatcagtactcaacccaaaaatatcatcactgccatcgcaagcctctgttatagtagcaccctgtaaaaactctctctctgcattatagttgtcctttcttgtagttaatttagttaatccagctgtgactccagaggtagagcaaggggctgggtctgtaacatgaaagctgatactagatatttccgcacaatttaaacgtctgggggatgaatacacgggttgtgtaggaagttcagaaacatctaatgcatttgcctggataggtacagaggataaagctgaagggtgtggccggtagatgacacttggtgaggtagtctgctcttgagttcctgattcatacacaccaagaaggtccggagaagtaggtgaagcaaggtttacttcatggaagccttccaagggatcattagccatagcaaaagcctcatcataagataacctgaagaacccaccgcggccgctgccggcgctcaggggcgctcacagagccgcagagagcgcgtcccgaagcagcgagaaacggaggaggacggcgagccctttccgctacactccacggcggcgggctcactacgccggcagccgccgagggaacgcgggactgcgcctgc

SEQ ID NO: 15978 - RNA, 6473 nt, Homo sapiens
  source 1..6473: mol_type = other RNA
gctgggattacaggcatgagccatcgcacctggccagtttttttttttttttttttttctaagtgcaatgggaagccactcaaagggctttaagcagggaagtgacattatctgattttcgttttataaagatccctgcggctgccgtcagtgattgtaggagggcaggagtggatgcaaggacagcagacattagtgcaggagttcaggtgaaagatgataatagcttgggcagagtggtagcagtggacatggagggaggtagacagatttaagatgtctcggagacagctgatggaatttgctgataactggaatgggagtgacaatgacaaataaaggaacctagaataagccccagaattttgcttaagcaactgagagttcagccatggcagatctgttaagcacaaaagttaaacacaaatacaaattcatactgcattggactcttttaagcagtgtcttatagaaaaaacattttatctagggaaaaatgcaacaacaaaaaccactgaaaacaaaagcctatgaataaaagcagacccgttttagactggatgcacaaaacaaaaacacacaggattcttgtggtggcgatgggagtaagtgaagacgtaacaggttgcaagttattttaaggactaagacccaatgttcagaaaccaaatcttgttcttccagtgtggatgcttagtcaaagactgtaaattgtcttcaagctgagagagaccatgaagagagaggagtggccacctaactaaccttcccagtttttgggagccaaacctagaccagaatgtaggtctaagtgactcccaatccagagctgtctccattaggccaggctctcaccccagctccaaaccaacttctaaaaacttgtccaagagtcctcctcttctttagaattggtaatcttggcaattaaattcagcgtagaaacactctcctgaacataatcagcatgctggttcttccttttctgttgccttgctcttcctaacagctcctcctttcgtctttgcaggctgcttctctgtcacaggaactcagggctcagtgctgtacttcatctccaaagtgtccctaaagcgcccatctgatcccatggctaactactccccaaattttctcctggactgaccttactgaatttagatttgtacatccaatacctgcttaacatatccactttgatgctcagtgggcacctcacacttgatctgtcaaacactgaatttctgtctctgttatgcacatacccaaactttccccaccatgtatttccccatctcaataaactgcaatagctcaagccaaaagcctaagattcagacctgaattctttcctttcctctctctcaaatgcaattcaacaattttcttaccttttattttttgttttggaatgaaggcacatataactgagctagtaataatgcttgattcataatacaccaccgatgttccatgcataactctcttattcatttgtccatgcatttattttgtttttgaatttttttaaaggggggcaaggtctacgttgcccaggttggaatatagtagctattcacaggtgaaatcatagcacactatagccttgaactggcctcaaggatcttcctatctcagactcccaagtagctgggactataagcacgcaccactacacccagctcatgtacttacttttaatgacaaatgaaccaccccaaaacccaccacctaacccagggactaaaacattaccagtgacttactcatagatttgctcctcctctacctctccagaggtaaccactatcttgaactttattactttttaaaagttttgtcacatatgtcaatgcctaaacagctgttcagttttagttgttcttgacttttataagaaaagtatcatgtcacatatagttttctcagaattgctttttcattctgagttattgtgctgcaagtagctggtattcattcattttgctgccatgtaataatcacccattctgtgaacacattacaccttcctaaaaatagacattttaatttattccagaacattcttatatgtgtgatctgggggacctgtgcaagcatttctcaagtatatactgaaaagtgaaattgctgacccatgggtatactttttttttttttttaaggtatgatcttactctgtcacccaaggtaagagtgcagtggcacaatcatgattcactgcagcctcaacctcctgggcttaagcaatccttccacctcagcttcccaagtagctgggaccacaggcatgcaccaccatgcccagctaattcaaaaaaatctttttgtgcagatgtggtctccctatgttgctcaagctggtcttgaactcttgggctcaagtgatcctcctaccttggcctcccaaagccaagaggcatgagccactgggcctggcccaacttttctagtgaatggtttttcacagtggatataccaattgatacccccatcagcaatatgtgagtgatcctaatgactaaaaccctctccaaaacttgactttgtgtttcttcattttcaccaatcgaatgaatttgaacatgtcattgtcatcttgatttacgttttcctgattgagagatgaaaacctcttaatgtttattggcccacatgcacttctaattgtgtggaaggcctggttcagtcttttgcctgtttttctgtgacactgtccttttttgttggtttgtagaatttctgcatacattcttgatactaagctattactagttataaatgttgcagatattgcctcacagtttgtagtttagctttagttttttttttagagacaaggtctccctatgttgcccaagttggacttgaacccctgggctcaagcaatcctcccacctcatcctcccaagttcatggacacagtgtgtgtgtgtgtgtgtgtgtgtgtgtgtgtgtaaatggagtttccctatttttcccaggcccgtctcaaactcctgggctcaagcagctcaagtaatccttctgcctctgcctcccaaagtgctgggattacaggcatgagccacaatgcctaactactgatgcacgatttctaaattaagaatttataatataccataacttatattcttttatggttatcttttatggtttttttttttcctgcttccagtttaagaagttcttcctaaagggagtaggatcaggaagataatcacattttctaaatatgtttcaatcacattttaatctataattccacatatagtttctacatcaagtcgtcatcctgttgcattaattttaaagagcatgcttctagtgtataaggttgaaaagcattcttccccttatagattactaaagatttattattaatgggtatactgattttctttagtcttactttttatttatcctttttaagtcatcaacaaactttttctgagtatttgattacctttctttcaaaccgtacagtatctcctggatttgtttctctttttatttaggtactttctccaaaagtgattttagtttgtacggaaaatcttctgaagctttgatggtacatattcttattaatgccctcacattagaataactattttcagaacataaaattgtaggttcaaagtttttttcaggttcaatttcacattcttgagctaggcatggtactgatggttttcaccataacatacaccaatgtccttttgtctgtgggctcccatccagcctggtggctgaagtcatctacaggtaagattgaccaaacctctgaacaggactgaaaaaaatgttatcttcagaaaaccagccctcttgtacactgctgctgtgaatacaaattgattaacttttctggatggcaatctagcaatgcagatcaaacatttaaaaatacatatatatctcgacacaattttatctccaggcatccacatgaaagaactccacaatgttcagaagtgtacagataaggatactcgtcacagcattataatatgaaaaataaactgaaaaccacctcatctccaaacacaattaaattatgttaaaattctataaacagggattaggatgtgtaggtttacccaagggaaaatatatttaatgtttaggtttaaaaagcaaaaaaaaagcctactttttgtttcaaaaatatgcatatgtaagtagaaaatatctgaaagctgaaaggctactatccaaaaatattaacagcagctttctctaaacagaaactaaagcagtttctcttttctttttgcttttctatacttattacatgtctaccacaaacctctttgttataatttctccagttgagtcagttttacaatttggaatgcagagatcaagtggttctataatcagcatatacttcgcacgtaccattcattcaatccacacccctttaaacccctttgacacacgtcaaactcatttacatctatgtccctccaatgacaatatagtggtcaacacatataaaacatgaatacactatatcaagacactcaggaatacatctctgggataaaatctgactgccttctattatattttaatgaataaccaaaataaagggattctttcagttacagagagcagaataattaaaatagtaactttcaaactttgtagcagcagaagtatttcttcaaataaaatcttttttgaaacccaatatagaaaacagataaaaataaagccattctagaggtgggggccttggaaagtgagtactatccactcagacttctttcttgcctctcacaaggaaggaagctactgtgtagtttgaaaattactatttaatacattctgctaaccctaaatgccatgtcagagctagaagagaaaatgtacacacattcaatctaacatttatttatttcaggttttttttttttttggcaactataaattacattcactagtacacctggaattcttcatagtgtgttcaactaaagaataagcaaacacagcatagatcagtttaaaagaaatcatggtacttcttagagcaatttgcaaaaggggaaaaaagtcttaggctcactccttggaaataaatatcaagtaaccataaaaatattcagccatttttcagttattcggggagttcaggcatggtcccacgcagagcatcagagttcctctttgaaataacccagctttgccaatgacatctcttttctcaactgcataacctcccaaaacatctgatcaacatcctgctgtttcacgagtccctgctgaatgtatcgaatgtatgtaaaaaagttacatacagaagtgatcctgtatctgcaaaaaggagaaatataataatagttgcttgagtcccctaatttaattctgtgtttacaggacttactctggccagtgagagcacattttctctttgcagtcttttacaattggctgtatcacactgaggtcctgatgactgccactcatagcactgcttgtgcttttatttcttgtatgcccctttttaaaaggtgtctttccacctggcaaaggctcctgcgtaggtgatgttggagaactggacaatacaagtgtcttcaatgcagctacttcagcttgaagtacatcaatttttccttgtgcttcttttagctgtttttctgctgttgcctgcttgatatttgcttctctcaccattttatgagcttcctcaaatagactagctgtgagttcttccaattcctgtccaagttgatctcgcacttttgaaagcctctcacattcttcatcttttaacttcagttccctctgagcttttgcgagttcttcttttaatcgttcatagcccttttctctaacttccaaaacagatgggcttcgtaaacgagacagactatcagtactcaacccaaaaatatcatcactgccatcgcaagcctctgttatagtagcaccctgtaaaaactctctctctgcattatagttgtcctttcttgtagttaatttagttaatccagctgtgactccagaggtagagcaaggggctgggtctgtaacatgaaagctgatactagatatttccgcacaatttaaacgtctgggggatgaatacacgggttgtgtaggaagttcagaaacatctaatgcatttgcctggataggtacagaggataaagctgaagggtgtggccggtagatgacacttggtgaggtagtctgctcttgagttcctgattcatacacaccaagaaggtccggagaagtaggtgaagcaaggtttacttcatggaagccttccaagggatcattagccatagcaaaagcctcatcataagataacctgagactccgcggccatatacaccttacgacgtgtgtgtgtgtggcgggagatgggaggggaggaatcctgtagaacccagatcccatcattccagcaactgccagagcgttcgagaatgtcatgtctgtacctgtcttct

SEQ ID NO: 15979 - RNA, 6882 nt, Homo sapiens
  source 1..6882: mol_type = other RNA
gctgggattacaggcatgagccatcgcacctggccagtttttttttttttttttttttctaagtgcaatgggaagccactcaaagggctttaagcagggaagtgacattatctgattttcgttttataaagatccctgcggctgccgtcagtgattgtaggagggcaggagtggatgcaaggacagcagacattagtgcaggagttcaggtgaaagatgataatagcttgggcagagtggtagcagtggacatggagggaggtagacagatttaagatgtctcggagacagctgatggaatttgctgataactggaatgggagtgacaatgacaaataaaggaacctagaataagccccagaattttgcttaagcaactgagagttcagccatggcagatctgttaagcacaaaagttaaacacaaatacaaattcatactgcattggactcttttaagcagtgtcttatagaaaaaacattttatctagggaaaaatgcaacaacaaaaaccactgaaaacaaaagcctatgaataaaagcagacccgttttagactggatgcacaaaacaaaaacacacaggattcttgtggtggcgatgggagtaagtgaagacgtaacaggttgcaagttattttaaggactaagacccaatgttcagaaaccaaatcttgttcttccagtgtggatgcttagtcaaagactgtaaattgtcttcaagctgagagagaccatgaagagagaggagtggccacctaactaaccttcccagtttttgggagccaaacctagaccagaatgtaggtctaagtgactcccaatccagagctgtctccattaggccaggctctcaccccagctccaaaccaacttctaaaaacttgtccaagagtcctcctcttctttagaattggtaatcttggcaattaaattcagcgtagaaacactctcctgaacataatcagcatgctggttcttccttttctgttgccttgctcttcctaacagctcctcctttcgtctttgcaggctgcttctctgtcacaggaactcagggctcagtgctgtacttcatctccaaagtgtccctaaagcgcccatctgatcccatggctaactactccccaaattttctcctggactgaccttactgaatttagatttgtacatccaatacctgcttaacatatccactttgatgctcagtgggcacctcacacttgatctgtcaaacactgaatttctgtctctgttatgcacatacccaaactttccccaccatgtatttccccatctcaataaactgcaatagctcaagccaaaagcctaagattcagacctgaattctttcctttcctctctctcaaatgcaattcaacaattttcttaccttttattttttgttttggaatgaaggcacatataactgagctagtaataatgcttgattcataatacaccaccgatgttccatgcataactctcttattcatttgtccatgcatttattttgtttttgaatttttttaaaggggggcaaggtctacgttgcccaggttggaatatagtagctattcacaggtgaaatcatagcacactatagccttgaactggcctcaaggatcttcctatctcagactcccaagtagctgggactataagcacgcaccactacacccagctcatgtacttacttttaatgacaaatgaaccaccccaaaacccaccacctaacccagggactaaaacattaccagtgacttactcatagatttgctcctcctctacctctccagaggtaaccactatcttgaactttattactttttaaaagttttgtcacatatgtcaatgcctaaacagctgttcagttttagttgttcttgacttttataagaaaagtatcatgtcacatatagttttctcagaattgctttttcattctgagttattgtgctgcaagtagctggtattcattcattttgctgccatgtaataatcacccattctgtgaacacattacaccttcctaaaaatagacattttaatttattccagaacattcttatatgtgtgatctgggggacctgtgcaagcatttctcaagtatatactgaaaagtgaaattgctgacccatgggtatactttttttttttttttaaggtatgatcttactctgtcacccaaggtaagagtgcagtggcacaatcatgattcactgcagcctcaacctcctgggcttaagcaatccttccacctcagcttcccaagtagctgggaccacaggcatgcaccaccatgcccagctaattcaaaaaaatctttttgtgcagatgtggtctccctatgttgctcaagctggtcttgaactcttgggctcaagtgatcctcctaccttggcctcccaaagccaagaggcatgagccactgggcctggcccaacttttctagtgaatggtttttcacagtggatataccaattgatacccccatcagcaatatgtgagtgatcctaatgactaaaaccctctccaaaacttgactttgtgtttcttcattttcaccaatcgaatgaatttgaacatgtcattgtcatcttgatttacgttttcctgattgagagatgaaaacctcttaatgtttattggcccacatgcacttctaattgtgtggaaggcctggttcagtcttttgcctgtttttctgtgacactgtccttttttgttggtttgtagaatttctgcatacattcttgatactaagctattactagttataaatgttgcagatattgcctcacagtttgtagtttagctttagttttttttttagagacaaggtctccctatgttgcccaagttggacttgaacccctgggctcaagcaatcctcccacctcatcctcccaagttcatggacacagtgtgtgtgtgtgtgtgtgtgtgtgtgtgtgtgtaaatggagtttccctatttttcccaggcccgtctcaaactcctgggctcaagcagctcaagtaatccttctgcctctgcctcccaaagtgctgggattacaggcatgagccacaatgcctaactactgatgcacgatttctaaattaagaatttataatataccataacttatattcttttatggttatcttttatggtttttttttttcctgcttccagtttaagaagttcttcctaaagggagtaggatcaggaagataatcacattttctaaatatgtttcaatcacattttaatctataattccacatatagtttctacatcaagtcgtcatcctgttgcattaattttaaagagcatgcttctagtgtataaggttgaaaagcattcttccccttatagattactaaagatttattattaatgggtatactgattttctttagtcttactttttatttatcctttttaagtcatcaacaaactttttctgagtatttgattacctttctttcaaaccgtacagtatctcctggatttgtttctctttttatttaggtactttctccaaaagtgattttagtttgtacggaaaatcttctgaagctttgatggtacatattcttattaatgccctcacattagaataactattttcagaacataaaattgtaggttcaaagtttttttcaggttcaatttcacattcttgagctaggcatggtactgatggttttcaccataacatacaccaatgtccttttgtctgtgggctcccatccagcctggtggctgaagtcatctacaggtaagattgaccaaacctctgaacaggactgaaaaaaatgttatcttcagaaaaccagccctcttgtacactgctgctgtgaatacaaattgattaacttttctggatggcaatctagcaatgcagatcaaacatttaaaaatacatatatatctcgacacaattttatctccaggcatccacatgaaagaactccacaatgttcagaagtgtacagataaggatactcgtcacagcattataatatgaaaaataaactgaaaaccacctcatctccaaacacaattaaattatgttaaaattctataaacagggattaggatgtgtaggtttacccaagggaaaatatatttaatgtttaggtttaaaaagcaaaaaaaaagcctactttttgtttcaaaaatatgcatatgtaagtagaaaatatctgaaagctgaaaggctactatccaaaaatattaacagcagctttctctaaacagaaactaaagcagtttctcttttctttttgcttttctatacttattacatgtctaccacaaacctctttgttataatttctccagttgagtcagttttacaatttggaatgcagagatcaagtggttctataatcagcatatacttcgcacgtaccattcattcaatccacacccctttaaacccctttgacacacgtcaaactcatttacatctatgtccctccaatgacaatatagtggtcaacacatataaaacatgaatacactatatcaagacactcaggaatacatctctgggataaaatctgactgccttctattatattttaatgaataaccaaaataaagggattctttcagttacagagagcagaataattaaaatagtaactttcaaactttgtagcagcagaagtatttcttcaaataaaatcttttttgaaacccaatatagaaaacagataaaaataaagccattctagaggtgggggccttggaaagtgagtactatccactcagacttctttcttgcctctcacaaggaaggaagctactgtgtagtttgaaaattactatttaatacattctgctaaccctaaatgccatgtcagagctagaagagaaaatgtacacacattcaatctaacatttatttatttcaggttttttttttttttggcaactataaattacattcactagtacacctggaattcttcatagtgtgttcaactaaagaataagcaaacacagcatagatcagtttaaaagaaatcatggtacttcttagagcaatttgcaaaaggggaaaaaagtcttaggctcactccttggaaataaatatcaagtaaccataaaaatattcagccatttttcagttattcggggagttcaggcatggtcccacgcagagcatcagagttcctctttgaaataacccagctttgccaatgacatctcttttctcaactgcataacctcccaaaacatctgatcaacatcctgctgtttcacgagtccctgctgaatgtatcgaatgtatgtaaaaaagttacatacagaagtgatcctgtatctgcaaaaaggagaaatataataatagttgcttgagtcccctaatttaattctgtgtttacaggacttactctggccagtgagagcacatttttttggtcctccgcattcaactgcagaagctttcacaaaccggataggttgtaatcccactggttcaatgcttagagtattgttttccacagcctccagaacagctgaagccaactcactttttgagaatgttaaacatggaaagatatcttcctggtagattttgtctaagaaaggacacgtcctgtccattgtgggctcatccttccacaatcggaattcattatacaaggataagtcagccagcatcatttttattgataattcgtcaaaatgcaattcaattaaaacaggttaacattggttattccatttaataaactcctggcttccatacaaaaatttaacaagcacacacatttcttcaagattaatgatggacttgaatttaacaatgtaaaagatggcttctctttgcagtcttttacaattggctgtatcacactgaggtcctgatgactgccactcatagcactgcttgtgcttttatttcttgtatgcccctttttaaaaggtgtctttccacctggcaaaggctcctgcgtaggtgatgttggagaactggacaatacaagtgtcttcaatgcagctacttcagcttgaagtacatcaatttttccttgtgcttcttttagctgtttttctgctgttgcctgcttgatatttgcttctctcaccattttatgagcttcctcaaatagactagctgtgagttcttccaattcctgtccaagttgatctcgcacttttgaaagcctctcacattcttcatcttttaacttcagttccctctgagcttttgcgagttcttcttttaatcgttcatagcccttttctctaacttccaaaacagatgggcttcgtaaacgagacagactatcagtactcaacccaaaaatatcatcactgccatcgcaagcctctgttatagtagcaccctgtaaaaactctctctctgcattatagttgtcctttcttgtagttaatttagttaatccagctgtgactccagaggtagagcaaggggctgggtctgtaacatgaaagctgatactagatatttccgcacaatttaaacgtctgggggatgaatacacgggttgtgtaggaagttcagaaacatctaatgcatttgcctggataggtacagaggataaagctgaagggtgtggccggtagatgacacttggtgaggtagtctgctcttgagttcctgattcatacacaccaagaaggtccggagaagtaggtgaagcaaggtttacttcatggaagccttccaagggatcattagccatagcaaaagcctcatcataagataacctgagactccgcggccatatacaccttacgacgtgtgtgtgtgtggcgggagatgggaggggaggaatcctgtagaacccagatcccatcattccagcaactgccagagcgttcgagaatgtcatgtctgtacctgtcttct

SEQ ID NO: 15980 - RNA, 9208 nt, Homo sapiens
  source 1..9208: mol_type = other RNA
gctgggattacaggcatgagccatcgcacctggccagtttttttttttttttttttttctaagtgcaatgggaagccactcaaagggctttaagcagggaagtgacattatctgattttcgttttataaagatccctgcggctgccgtcagtgattgtaggagggcaggagtggatgcaaggacagcagacattagtgcaggagttcaggtgaaagatgataatagcttgggcagagtggtagcagtggacatggagggaggtagacagatttaagatgtctcggagacagctgatggaatttgctgataactggaatgggagtgacaatgacaaataaaggaacctagaataagccccagaattttgcttaagcaactgagagttcagccatggcagatctgttaagcacaaaagttaaacacaaatacaaattcatactgcattggactcttttaagcagtgtcttatagaaaaaacattttatctagggaaaaatgcaacaacaaaaaccactgaaaacaaaagcctatgaataaaagcagacccgttttagactggatgcacaaaacaaaaacacacaggattcttgtggtggcgatgggagtaagtgaagacgtaacaggttgcaagttattttaaggactaagacccaatgttcagaaaccaaatcttgttcttccagtgtggatgcttagtcaaagactgtaaattgtcttcaagctgagagagaccatgaagagagaggagtggccacctaactaaccttcccagtttttgggagccaaacctagaccagaatgtaggtctaagtgactcccaatccagagctgtctccattaggccaggctctcaccccagctccaaaccaacttctaaaaacttgtccaagagtcctcctcttctttagaattggtaatcttggcaattaaattcagcgtagaaacactctcctgaacataatcagcatgctggttcttccttttctgttgccttgctcttcctaacagctcctcctttcgtctttgcaggctgcttctctgtcacaggaactcagggctcagtgctgtacttcatctccaaagtgtccctaaagcgcccatctgatcccatggctaactactccccaaattttctcctggactgaccttactgaatttagatttgtacatccaatacctgcttaacatatccactttgatgctcagtgggcacctcacacttgatctgtcaaacactgaatttctgtctctgttatgcacatacccaaactttccccaccatgtatttccccatctcaataaactgcaatagctcaagccaaaagcctaagattcagacctgaattctttcctttcctctctctcaaatgcaattcaacaattttcttaccttttattttttgttttggaatgaaggcacatataactgagctagtaataatgcttgattcataatacaccaccgatgttccatgcataactctcttattcatttgtccatgcatttattttgtttttgaatttttttaaaggggggcaaggtctacgttgcccaggttggaatatagtagctattcacaggtgaaatcatagcacactatagccttgaactggcctcaaggatcttcctatctcagactcccaagtagctgggactataagcacgcaccactacacccagctcatgtacttacttttaatgacaaatgaaccaccccaaaacccaccacctaacccagggactaaaacattaccagtgacttactcatagatttgctcctcctctacctctccagaggtaaccactatcttgaactttattactttttaaaagttttgtcacatatgtcaatgcctaaacagctgttcagttttagttgttcttgacttttataagaaaagtatcatgtcacatatagttttctcagaattgctttttcattctgagttattgtgctgcaagtagctggtattcattcattttgctgccatgtaataatcacccattctgtgaacacattacaccttcctaaaaatagacattttaatttattccagaacattcttatatgtgtgatctgggggacctgtgcaagcatttctcaagtatatactgaaaagtgaaattgctgacccatgggtatactttttttttttttttaaggtatgatcttactctgtcacccaaggtaagagtgcagtggcacaatcatgattcactgcagcctcaacctcctgggcttaagcaatccttccacctcagcttcccaagtagctgggaccacaggcatgcaccaccatgcccagctaattcaaaaaaatctttttgtgcagatgtggtctccctatgttgctcaagctggtcttgaactcttgggctcaagtgatcctcctaccttggcctcccaaagccaagaggcatgagccactgggcctggcccaacttttctagtgaatggtttttcacagtggatataccaattgatacccccatcagcaatatgtgagtgatcctaatgactaaaaccctctccaaaacttgactttgtgtttcttcattttcaccaatcgaatgaatttgaacatgtcattgtcatcttgatttacgttttcctgattgagagatgaaaacctcttaatgtttattggcccacatgcacttctaattgtgtggaaggcctggttcagtcttttgcctgtttttctgtgacactgtccttttttgttggtttgtagaatttctgcatacattcttgatactaagctattactagttataaatgttgcagatattgcctcacagtttgtagtttagctttagttttttttttagagacaaggtctccctatgttgcccaagttggacttgaacccctgggctcaagcaatcctcccacctcatcctcccaagttcatggacacagtgtgtgtgtgtgtgtgtgtgtgtgtgtgtgtgtaaatggagtttccctatttttcccaggcccgtctcaaactcctgggctcaagcagctcaagtaatccttctgcctctgcctcccaaagtgctgggattacaggcatgagccacaatgcctaactactgatgcacgatttctaaattaagaatttataatataccataacttatattcttttatggttatcttttatggtttttttttttcctgcttccagtttaagaagttcttcctaaagggagtaggatcaggaagataatcacattttctaaatatgtttcaatcacattttaatctataattccacatatagtttctacatcaagtcgtcatcctgttgcattaattttaaagagcatgcttctagtgtataaggttgaaaagcattcttccccttatagattactaaagatttattattaatgggtatactgattttctttagtcttactttttatttatcctttttaagtcatcaacaaactttttctgagtatttgattacctttctttcaaaccgtacagtatctcctggatttgtttctctttttatttaggtactttctccaaaagtgattttagtttgtacggaaaatcttctgaagctttgatggtacatattcttattaatgccctcacattagaataactattttcagaacataaaattgtaggttcaaagtttttttcaggttcaatttcacattcttgagctaggcatggtactgatggttttcaccataacatacaccaatgtccttttgtctgtgggctcccatccagcctggtggctgaagtcatctacaggtaagattgaccaaacctctgaacaggactgaaaaaaatgttatcttcagaaaaccagccctcttgtacactgctgctgtgaatacaaattgattaacttttctggatggcaatctagcaatgcagatcaaacatttaaaaatacatatatatctcgacacaattttatctccaggcatccacatgaaagaactccacaatgttcagaagtgtacagataaggatactcgtcacagcattataatatgaaaaataaactgaaaaccacctcatctccaaacacaattaaattatgttaaaattctataaacagggattaggatgtgtaggtttacccaagggaaaatatatttaatgtttaggtttaaaaagcaaaaaaaaagcctactttttgtttcaaaaatatgcatatgtaagtagaaaatatctgaaagctgaaaggctactatccaaaaatattaacagcagctttctctaaacagaaactaaagcagtttctcttttctttttgcttttctatacttattacatgtctaccacaaacctctttgttataatttctccagttgagtcagttttacaatttggaatgcagagatcaagtggttctataatcagcatatacttcgcacgtaccattcattcaatccacacccctttaaacccctttgacacacgtcaaactcatttacatctatgtccctccaatgacaatatagtggtcaacacatataaaacatgaatacactatatcaagacactcaggaatacatctctgggataaaatctgactgccttctattatattttaatgaataaccaaaataaagggattctttcagttacagagagcagaataattaaaatagtaactttcaaactttgtagcagcagaagtatttcttcaaataaaatcttttttgaaacccaatatagaaaacagataaaaataaagccattctagaggtgggggccttggaaagtgagtactatccactcagacttctttcttgcctctcacaaggaaggaagctactgtgtagtttgaaaattactatttaatacattctgctaaccctaaatgccatgtcagagctagaagagaaaatgtacacacattcaatctaacatttatttatttcaggttttttttttttttggcaactataaattacattcactagtacacctggaattcttcatagtgtgttcaactaaagaataagcaaacacagcatagatcagtttaaaagaaatcatggtacttcttagagcaatttgcaaaaggggaaaaaagtcttaggctcactccttggaaataaatatcaagtaaccataaaaatattcagccatttttcagttattcggggagttcaggcatggtcccacgcagagcatcagagttcctctttgaaataacccagctttgccaatgacatctcttttctcaactgcataacctcccaaaacatctgatcaacatcctgctgtttcacgagtccctgctgaatgtatcgaatgtatgtaaaaaagttacatacagaagtgatcctgtatctgcaaaaaggagaaatataataatagttgcttgagtcccctaatttaattctgtgtttacaggacttactctggccagtgagagcacatttttttggtcctccgcattcaactgcagaagctttcacaaaccggataggttgtaatcccactggttcaatgcttagagtattgttttccacagcctccagaacagctgaagccaactcactttttgagaatgttaaacatggaaagatatcttcctggtagattttgtctaagaaaggacacgtcctgtccattgtgggctcatccttccacaatcggaattcattatacaaggataagtcagcctctttgcagtcttttacaattggctgtatcacactgaggtcctgatgactgccactcatagcactgcttgtgcttttatttcttgtatgcccctttttaaaaggtgtctttccacctggcaaaggctcctgcgtaggtgatgttggagaactggacaatacaagtgtcttcaatgcagctacttcagcttgaagtacatcaatttttccttgtgcttcttttagctgtttttctgctgttgcctgcttgatatttgcttctctcaccattttatgagcttccattgtatcacaagtgccaacagtattcagtatagtaacatgttgtacaggtttgtagcccaggagcaataagcaatatcatatagccaaggtgtgtaataggctgtaccatctaggttttaccacatcttggtttgtgtaagtatattctaccgatttctgcacgatgaaatcaaaactgtgcatattgagtttattcagaataatctttaattcctaaaaagatatgcaaacacacacatataaagtgcaaaaaaagaatcttttcataagacaatggtaaacagatcatgaaggcacaattaagaccaaataaaaactttgagcgctttttccacgattcataaataattggttcgaatacaactttcttcattaccaaaatcatctttaatcaatgtactttgttttccagaaagtagccacagtgtcaatgctaacagccaccactgggttagaaaaggttagagactccaaactatattttttagatatgctttttcacttattgcctattgcctaagctgcatttctggcccttcacatcctgctacttacagggagaagtttctttctgttttttctacttctatttcatgtaacagaacatacatacatgtgcagatgggtgaaactaagcagggctagctaaattaaatgcaagtagtcaggaaatcaaaattaacataaatagcttaatatatttgctttcttacctaatatccatatcactacaaaattttcttccagtcagacaatactggaagaaaaatctaatgcttctgtataaccttctattcagaaatgtaacaagtcacatagcttctattctagctctttaactttccactcttcctatccttaaatttattctcctctcatctctgatgactagctagctaaataaataaacagattaattttaaaatgttcatgaaagaaaatgaccccaaaaagacagaaaagaaggcaaaggggtatggagcagagaaggcatggaaagccctacatgtctaaagacattcagggcaatgttacttgtaatgataaaagttgtggaacaggcacctagtagattatgactatcgttacaattagtgatggtgcagcaacattaaaaatgttatttagaaaaacacaaaatattaaattacaactaagtaagaatacatacatacctgagactgtgaaatagattatgaataaataataacaaaaggtgatggaatttccacccccccaagtttattataataaaagttttaagaacaaatctttaggaaaaaaacatatatatatcgttaaatgataatggcattagccattccagtaacacatcaatgtttttgttaaggaacttctaaagactcaaggtcttaacccaaaggagacactttacagcaacagttcttactcatggaagtactaccctcacctcacccccaggggtatctgtatgctgtcaaaatgaccgggggtattaccagcacttttctgagcaaagcctattataatggtttattgtgtacgtcaacttgactgaatcaaagggtgctcgaatatgtagtcaaacattatcctgaatgtttctggataagaataacatttacattggtagactgagtaaagtagactgccctctagaatgtgggtgaccctcatccaatcagttgatggcctgaatagaacaaaaaagggtgccgctccctcaaggaagagattttttttctgccttcagactcaaactgaaacatttgctcttcccagttctcagaccttcaaagttggactggaagtgcaccatcagccctcctgggcctccagtttgctgactcccactgcagctccctgggacttgccagcctccataacagcaagagccaactccctataataatgagtgcctctgtccctctctctccctctctgtatctctctatacatgtatatgtatataggctctgtttttctggagaaccctgactaaaacaccaaggacactaaacgtcctacagtgttagtggcacccctatggagaaacactgctccagttaggtagaaatttttcctggtggcgggctggatataaaaagtatgccttcttacaagtagatgtgccttctaacatttctcaaatcatcccatgtaagatgactatctcaaagagtttgccctcttagttgtacagtcatatgtagttaatctaaagtagcccgtaaatacttggtaaaataaaaatcaatactaaaatttgcctcctttctttgcacacatacatttttaaataatctgatactggtggcccatagatgttttttatttcttttcacatcatcttaagttgtaaactctacattgcttaaagatttctcttttgcttagaggacttataaatatacatgaagctaagcaaatatttttcaagattccctcaaaatacaattttgtcaatatataaaagtcaagatgttgctgttggccaagatgtaaatagaccaacctcaaatagactagctgtgagttcttccaattcctgtccaagttgatctcgcacttttgaaagcctctcacattcttcatcttttaacttcagttccctctgagcttttgcgagttcttcttttaatcgttcatagcccttttctctaacttccaaaacagatgggcttcgtaaacgagacagactatcagtactcaacccaaaaatatcatcactgccatcgcaagcctctgttatagtagcaccctgtaaaaactctctctctgcattatagttgtcctttcttgtagttaatttagttaatccagctgtgactccagaggtagagcaaggggctgggtctgtaacatgaaagctgatactagatatttccgcacaatttaaacgtctgggggatgaatacacgggttgtgtaggaagttcagaaacatctaatgcatttgcctggataggtacagaggataaagctgaagggtgtggccggtagatgacacttggtgaggtagtctgctcttgagttcctgattcatacacaccaagaaggtccggagaagtaggtgaagcaaggtttacttcatggaagccttccaagggatcattagccatagcaaaagcctcatcataagataacctgaagaacccaccgcggccgctgccggcgctcaggggcgctcacagagccgcagagagcgcgtcccgaagcagcgagaaacggaggaggacggcgagccctttccgctacactccacggcggcgggctcactac

SEQ ID NO: 15981 - RNA, 6823 nt, Homo sapiens
  source 1..6823: mol_type = other RNA
gctgggattacaggcatgagccatcgcacctggccagtttttttttttttttttttttctaagtgcaatgggaagccactcaaagggctttaagcagggaagtgacattatctgattttcgttttataaagatccctgcggctgccgtcagtgattgtaggagggcaggagtggatgcaaggacagcagacattagtgcaggagttcaggtgaaagatgataatagcttgggcagagtggtagcagtggacatggagggaggtagacagatttaagatgtctcggagacagctgatggaatttgctgataactggaatgggagtgacaatgacaaataaaggaacctagaataagccccagaattttgcttaagcaactgagagttcagccatggcagatctgttaagcacaaaagttaaacacaaatacaaattcatactgcattggactcttttaagcagtgtcttatagaaaaaacattttatctagggaaaaatgcaacaacaaaaaccactgaaaacaaaagcctatgaataaaagcagacccgttttagactggatgcacaaaacaaaaacacacaggattcttgtggtggcgatgggagtaagtgaagacgtaacaggttgcaagttattttaaggactaagacccaatgttcagaaaccaaatcttgttcttccagtgtggatgcttagtcaaagactgtaaattgtcttcaagctgagagagaccatgaagagagaggagtggccacctaactaaccttcccagtttttgggagccaaacctagaccagaatgtaggtctaagtgactcccaatccagagctgtctccattaggccaggctctcaccccagctccaaaccaacttctaaaaacttgtccaagagtcctcctcttctttagaattggtaatcttggcaattaaattcagcgtagaaacactctcctgaacataatcagcatgctggttcttccttttctgttgccttgctcttcctaacagctcctcctttcgtctttgcaggctgcttctctgtcacaggaactcagggctcagtgctgtacttcatctccaaagtgtccctaaagcgcccatctgatcccatggctaactactccccaaattttctcctggactgaccttactgaatttagatttgtacatccaatacctgcttaacatatccactttgatgctcagtgggcacctcacacttgatctgtcaaacactgaatttctgtctctgttatgcacatacccaaactttccccaccatgtatttccccatctcaataaactgcaatagctcaagccaaaagcctaagattcagacctgaattctttcctttcctctctctcaaatgcaattcaacaattttcttaccttttattttttgttttggaatgaaggcacatataactgagctagtaataatgcttgattcataatacaccaccgatgttccatgcataactctcttattcatttgtccatgcatttattttgtttttgaatttttttaaaggggggcaaggtctacgttgcccaggttggaatatagtagctattcacaggtgaaatcatagcacactatagccttgaactggcctcaaggatcttcctatctcagactcccaagtagctgggactataagcacgcaccactacacccagctcatgtacttacttttaatgacaaatgaaccaccccaaaacccaccacctaacccagggactaaaacattaccagtgacttactcatagatttgctcctcctctacctctccagaggtaaccactatcttgaactttattactttttaaaagttttgtcacatatgtcaatgcctaaacagctgttcagttttagttgttcttgacttttataagaaaagtatcatgtcacatatagttttctcagaattgctttttcattctgagttattgtgctgcaagtagctggtattcattcattttgctgccatgtaataatcacccattctgtgaacacattacaccttcctaaaaatagacattttaatttattccagaacattcttatatgtgtgatctgggggacctgtgcaagcatttctcaagtatatactgaaaagtgaaattgctgacccatgggtatactttttttttttttttaaggtatgatcttactctgtcacccaaggtaagagtgcagtggcacaatcatgattcactgcagcctcaacctcctgggcttaagcaatccttccacctcagcttcccaagtagctgggaccacaggcatgcaccaccatgcccagctaattcaaaaaaatctttttgtgcagatgtggtctccctatgttgctcaagctggtcttgaactcttgggctcaagtgatcctcctaccttggcctcccaaagccaagaggcatgagccactgggcctggcccaacttttctagtgaatggtttttcacagtggatataccaattgatacccccatcagcaatatgtgagtgatcctaatgactaaaaccctctccaaaacttgactttgtgtttcttcattttcaccaatcgaatgaatttgaacatgtcattgtcatcttgatttacgttttcctgattgagagatgaaaacctcttaatgtttattggcccacatgcacttctaattgtgtggaaggcctggttcagtcttttgcctgtttttctgtgacactgtccttttttgttggtttgtagaatttctgcatacattcttgatactaagctattactagttataaatgttgcagatattgcctcacagtttgtagtttagctttagttttttttttagagacaaggtctccctatgttgcccaagttggacttgaacccctgggctcaagcaatcctcccacctcatcctcccaagttcatggacacagtgtgtgtgtgtgtgtgtgtgtgtgtgtgtgtgtaaatggagtttccctatttttcccaggcccgtctcaaactcctgggctcaagcagctcaagtaatccttctgcctctgcctcccaaagtgctgggattacaggcatgagccacaatgcctaactactgatgcacgatttctaaattaagaatttataatataccataacttatattcttttatggttatcttttatggtttttttttttcctgcttccagtttaagaagttcttcctaaagggagtaggatcaggaagataatcacattttctaaatatgtttcaatcacattttaatctataattccacatatagtttctacatcaagtcgtcatcctgttgcattaattttaaagagcatgcttctagtgtataaggttgaaaagcattcttccccttatagattactaaagatttattattaatgggtatactgattttctttagtcttactttttatttatcctttttaagtcatcaacaaactttttctgagtatttgattacctttctttcaaaccgtacagtatctcctggatttgtttctctttttatttaggtactttctccaaaagtgattttagtttgtacggaaaatcttctgaagctttgatggtacatattcttattaatgccctcacattagaataactattttcagaacataaaattgtaggttcaaagtttttttcaggttcaatttcacattcttgagctaggcatggtactgatggttttcaccataacatacaccaatgtccttttgtctgtgggctcccatccagcctggtggctgaagtcatctacaggtaagattgaccaaacctctgaacaggactgaaaaaaatgttatcttcagaaaaccagccctcttgtacactgctgctgtgaatacaaattgattaacttttctggatggcaatctagcaatgcagatcaaacatttaaaaatacatatatatctcgacacaattttatctccaggcatccacatgaaagaactccacaatgttcagaagtgtacagataaggatactcgtcacagcattataatatgaaaaataaactgaaaaccacctcatctccaaacacaattaaattatgttaaaattctataaacagggattaggatgtgtaggtttacccaagggaaaatatatttaatgtttaggtttaaaaagcaaaaaaaaagcctactttttgtttcaaaaatatgcatatgtaagtagaaaatatctgaaagctgaaaggctactatccaaaaatattaacagcagctttctctaaacagaaactaaagcagtttctcttttctttttgcttttctatacttattacatgtctaccacaaacctctttgttataatttctccagttgagtcagttttacaatttggaatgcagagatcaagtggttctataatcagcatatacttcgcacgtaccattcattcaatccacacccctttaaacccctttgacacacgtcaaactcatttacatctatgtccctccaatgacaatatagtggtcaacacatataaaacatgaatacactatatcaagacactcaggaatacatctctgggataaaatctgactgccttctattatattttaatgaataaccaaaataaagggattctttcagttacagagagcagaataattaaaatagtaactttcaaactttgtagcagcagaagtatttcttcaaataaaatcttttttgaaacccaatatagaaaacagataaaaataaagccattctagaggtgggggccttggaaagtgagtactatccactcagacttctttcttgcctctcacaaggaaggaagctactgtgtagtttgaaaattactatttaatacattctgctaaccctaaatgccatgtcagagctagaagagaaaatgtacacacattcaatctaacatttatttatttcaggttttttttttttttggcaactataaattacattcactagtacacctggaattcttcatagtgtgttcaactaaagaataagcaaacacagcatagatcagtttaaaagaaatcatggtacttcttagagcaatttgcaaaaggggaaaaaagtcttaggctcactccttggaaataaatatcaagtaaccataaaaatattcagccatttttcagttattcggggagttcaggcatggtcccacgcagagcatcagagttcctctttgaaataacccagctttgccaatgacatctcttttctcaactgcataacctcccaaaacatctgatcaacatcctgctgtttcacgagtccctgctgaatgtatcgaatgtatgtaaaaaagttacatacagaagtgatcctgtatctgcaaaaaggagaaatataataatagttgcttgagtcccctaatttaattctgtgtttacaggacttactctggccagtgagagcacatttttttggtcctccgcattcaactgcagaagctttcacaaaccggataggttgtaatcccactggttcaatgcttagagtattgttttccacagcctccagaacagctgaagccaactcactttttgagaatgttaaacatggaaagatatcttcctggtagattttgtctaagaaaggacacgtcctgtccattgtgggctcatccttccacaatcggaattcattatacaaggataagtcagcctctttgcagtcttttacaattggctgtatcacactgaggtcctgatgactgccactcatagcactgcttgtgcttttatttcttgtatgcccctttttaaaaggtgtctttccacctggcaaaggctcctgcgtaggtgatgttggagaactggacaatacaagtgtcttcaatgcagctacttcagcttgaagtacatcaatttttccttgtgcttcttttagctgtttttctgctgttgcctgcttgatatttgcttctctcaccattttatgagcttccattgtatcacaagtgccaacagtattcagtatagtaacatgttgtacaggtttgtagcccaggagcaataagcaatatcatatagccaaggtgtgtaataggctgtaccatctaggttttaccacatcttggtttgtgtaagtatattctaccgatttctgcacgatgaaatctcaaatagactagctgtgagttcttccaattcctgtccaagttgatctcgcacttttgaaagcctctcacattcttcatcttttaacttcagttccctctgagcttttgcgagttcttcttttaatcgttcatagcccttttctctaacttccaaaacagatgggcttcgtaaacgagacagactatcagtactcaacccaaaaatatcatcactgccatcgcaagcctctgttatagtagcaccctgtaaaaactctctctctgcattatagttgtcctttcttgtagttaatttagttaatccagctgtgactccagaggtagagcaaggggctgggtctgtaacatgaaagctgatactagatatttccgcacaatttaaacgtctgggggatgaatacacgggttgtgtaggaagttcagaaacatctaatgcatttgccaagaaggtccggagaagtaggtgaagcaaggtttacttcatggaagccttccaagggatcattagccatagcaaaagcctcatcataagataacctgaagaacccaccgcggccgctgccggcgctcaggggcgctcacagagccgcagagagcgcgtcccgaagcagcgagaaacggaggaggacggcgagccctttccgctacactccacggcggcgggctcactacgccggcagccgccgagggaacgcgggactgcgcc

SEQ ID NO: 15982 - RNA, 6961 nt, Homo sapiens
  source 1..6961: mol_type = other RNA
gctgggattacaggcatgagccatcgcacctggccagtttttttttttttttttttttctaagtgcaatgggaagccactcaaagggctttaagcagggaagtgacattatctgattttcgttttataaagatccctgcggctgccgtcagtgattgtaggagggcaggagtggatgcaaggacagcagacattagtgcaggagttcaggtgaaagatgataatagcttgggcagagtggtagcagtggacatggagggaggtagacagatttaagatgtctcggagacagctgatggaatttgctgataactggaatgggagtgacaatgacaaataaaggaacctagaataagccccagaattttgcttaagcaactgagagttcagccatggcagatctgttaagcacaaaagttaaacacaaatacaaattcatactgcattggactcttttaagcagtgtcttatagaaaaaacattttatctagggaaaaatgcaacaacaaaaaccactgaaaacaaaagcctatgaataaaagcagacccgttttagactggatgcacaaaacaaaaacacacaggattcttgtggtggcgatgggagtaagtgaagacgtaacaggttgcaagttattttaaggactaagacccaatgttcagaaaccaaatcttgttcttccagtgtggatgcttagtcaaagactgtaaattgtcttcaagctgagagagaccatgaagagagaggagtggccacctaactaaccttcccagtttttgggagccaaacctagaccagaatgtaggtctaagtgactcccaatccagagctgtctccattaggccaggctctcaccccagctccaaaccaacttctaaaaacttgtccaagagtcctcctcttctttagaattggtaatcttggcaattaaattcagcgtagaaacactctcctgaacataatcagcatgctggttcttccttttctgttgccttgctcttcctaacagctcctcctttcgtctttgcaggctgcttctctgtcacaggaactcagggctcagtgctgtacttcatctccaaagtgtccctaaagcgcccatctgatcccatggctaactactccccaaattttctcctggactgaccttactgaatttagatttgtacatccaatacctgcttaacatatccactttgatgctcagtgggcacctcacacttgatctgtcaaacactgaatttctgtctctgttatgcacatacccaaactttccccaccatgtatttccccatctcaataaactgcaatagctcaagccaaaagcctaagattcagacctgaattctttcctttcctctctctcaaatgcaattcaacaattttcttaccttttattttttgttttggaatgaaggcacatataactgagctagtaataatgcttgattcataatacaccaccgatgttccatgcataactctcttattcatttgtccatgcatttattttgtttttgaatttttttaaaggggggcaaggtctacgttgcccaggttggaatatagtagctattcacaggtgaaatcatagcacactatagccttgaactggcctcaaggatcttcctatctcagactcccaagtagctgggactataagcacgcaccactacacccagctcatgtacttacttttaatgacaaatgaaccaccccaaaacccaccacctaacccagggactaaaacattaccagtgacttactcatagatttgctcctcctctacctctccagaggtaaccactatcttgaactttattactttttaaaagttttgtcacatatgtcaatgcctaaacagctgttcagttttagttgttcttgacttttataagaaaagtatcatgtcacatatagttttctcagaattgctttttcattctgagttattgtgctgcaagtagctggtattcattcattttgctgccatgtaataatcacccattctgtgaacacattacaccttcctaaaaatagacattttaatttattccagaacattcttatatgtgtgatctgggggacctgtgcaagcatttctcaagtatatactgaaaagtgaaattgctgacccatgggtatactttttttttttttttaaggtatgatcttactctgtcacccaaggtaagagtgcagtggcacaatcatgattcactgcagcctcaacctcctgggcttaagcaatccttccacctcagcttcccaagtagctgggaccacaggcatgcaccaccatgcccagctaattcaaaaaaatctttttgtgcagatgtggtctccctatgttgctcaagctggtcttgaactcttgggctcaagtgatcctcctaccttggcctcccaaagccaagaggcatgagccactgggcctggcccaacttttctagtgaatggtttttcacagtggatataccaattgatacccccatcagcaatatgtgagtgatcctaatgactaaaaccctctccaaaacttgactttgtgtttcttcattttcaccaatcgaatgaatttgaacatgtcattgtcatcttgatttacgttttcctgattgagagatgaaaacctcttaatgtttattggcccacatgcacttctaattgtgtggaaggcctggttcagtcttttgcctgtttttctgtgacactgtccttttttgttggtttgtagaatttctgcatacattcttgatactaagctattactagttataaatgttgcagatattgcctcacagtttgtagtttagctttagttttttttttagagacaaggtctccctatgttgcccaagttggacttgaacccctgggctcaagcaatcctcccacctcatcctcccaagttcatggacacagtgtgtgtgtgtgtgtgtgtgtgtgtgtgtgtgtaaatggagtttccctatttttcccaggcccgtctcaaactcctgggctcaagcagctcaagtaatccttctgcctctgcctcccaaagtgctgggattacaggcatgagccacaatgcctaactactgatgcacgatttctaaattaagaatttataatataccataacttatattcttttatggttatcttttatggtttttttttttcctgcttccagtttaagaagttcttcctaaagggagtaggatcaggaagataatcacattttctaaatatgtttcaatcacattttaatctataattccacatatagtttctacatcaagtcgtcatcctgttgcattaattttaaagagcatgcttctagtgtataaggttgaaaagcattcttccccttatagattactaaagatttattattaatgggtatactgattttctttagtcttactttttatttatcctttttaagtcatcaacaaactttttctgagtatttgattacctttctttcaaaccgtacagtatctcctggatttgtttctctttttatttaggtactttctccaaaagtgattttagtttgtacggaaaatcttctgaagctttgatggtacatattcttattaatgccctcacattagaataactattttcagaacataaaattgtaggttcaaagtttttttcaggttcaatttcacattcttgagctaggcatggtactgatggttttcaccataacatacaccaatgtccttttgtctgtgggctcccatccagcctggtggctgaagtcatctacaggtaagattgaccaaacctctgaacaggactgaaaaaaatgttatcttcagaaaaccagccctcttgtacactgctgctgtgaatacaaattgattaacttttctggatggcaatctagcaatgcagatcaaacatttaaaaatacatatatatctcgacacaattttatctccaggcatccacatgaaagaactccacaatgttcagaagtgtacagataaggatactcgtcacagcattataatatgaaaaataaactgaaaaccacctcatctccaaacacaattaaattatgttaaaattctataaacagggattaggatgtgtaggtttacccaagggaaaatatatttaatgtttaggtttaaaaagcaaaaaaaaagcctactttttgtttcaaaaatatgcatatgtaagtagaaaatatctgaaagctgaaaggctactatccaaaaatattaacagcagctttctctaaacagaaactaaagcagtttctcttttctttttgcttttctatacttattacatgtctaccacaaacctctttgttataatttctccagttgagtcagttttacaatttggaatgcagagatcaagtggttctataatcagcatatacttcgcacgtaccattcattcaatccacacccctttaaacccctttgacacacgtcaaactcatttacatctatgtccctccaatgacaatatagtggtcaacacatataaaacatgaatacactatatcaagacactcaggaatacatctctgggataaaatctgactgccttctattatattttaatgaataaccaaaataaagggattctttcagttacagagagcagaataattaaaatagtaactttcaaactttgtagcagcagaagtatttcttcaaataaaatcttttttgaaacccaatatagaaaacagataaaaataaagccattctagaggtgggggccttggaaagtgagtactatccactcagacttctttcttgcctctcacaaggaaggaagctactgtgtagtttgaaaattactatttaatacattctgctaaccctaaatgccatgtcagagctagaagagaaaatgtacacacattcaatctaacatttatttatttcaggttttttttttttttggcaactataaattacattcactagtacacctggaattcttcatagtgtgttcaactaaagaataagcaaacacagcatagatcagtttaaaagaaatcatggtacttcttagagcaatttgcaaaaggggaaaaaagtcttaggctcactccttggaaataaatatcaagtaaccataaaaatattcagccatttttcagttattcggggagttcaggcatggtcccacgcagagcatcagagttcctctttgaaataacccagctttgccaatgacatctcttttctcaactgcataacctcccaaaacatctgatcaacatcctgctgtttcacgagtccctgctgaatgtatcgaatgtatgtaaaaaagttacatacagaagtgatcctgtatctgcaaaaaggagaaatataataatagttgcttgagtcccctaatttaattctgtgtttacaggacttactctggccagtgagagcacatttttttggtcctccgcattcaactgcagaagctttcacaaaccggataggttgtaatcccactggttcaatgcttagagtattgttttccacagcctccagaacagctgaagccaactcactttttgagaatgttaaacatggaaagatatcttcctggtagattttgtctaagaaaggacacgtcctgtccattgtgggctcatccttccacaatcggaattcattatacaaggataagtcagcctctttgcagtcttttacaattggctgtatcacactgaggtcctgatgactgccactcatagcactgcttgtgcttttatttcttgtatgcccctttttaaaaggtgtctttccacctggcaaaggctcctgcgtaggtgatgttggagaactggacaatacaagtgtcttcaatgcagctacttcagcttgaagtacatcaatttttccttgtgcttcttttagctgtttttctgctgttgcctgcttgatatttgcttctctcaccattttatgagcttcctcaaatagactagctgtgagttcttccaattcctgtccaagttgatctcgcacttttgaaagcctctcacattcttcatcttttaacttcagttccctctgagcttttgcgagttcttcttttaatcgttcatagcccttttctctaacttccaaaacagatgggcttcgtaaacgagacagactatcagtactcaacccaaaaatatcatcactgccatcgcaagcctctgttatagtagcaccctgtaaaaactctctctctgcattatagttgtcctttcttgtagttaatttagttaatccagctgtgactccagaggtagagcaaggggctgggtctgtaacatgaaagctgatactagatatttccgcacaatttaaacgtctgggggatgaatacacgggttgtgtaggaagttcagaaacatctaatgcatttgccaagaaggtccggagaagtaggtgaagcaaggtttacttcatggaagccttccaagggatcattagccatagcaaaagcctcatcataagataaccctttcatcttttttaatcccataacaaccggcaactcttcacatgctgcgacttccacccagcatcatcacttctggagccagtaagctcgcgcttcctgggcggtcggggcgagttgtcaacgctgggagggcagagccatgcaatcccacccgtgcagttcgtctcaactcccccgaacacaagtctggcggcacggagctgcctacttgggcgcgactccgggcgcctgcccggaatttcccaccaggtttcaccgaaacctcccgagggtgacctctacgcctcagcacggtgcctcgcgcgtagtttcctaagactgggacacgaaaccaccccaggtccacagccctgccgcgcggcgtccggtgttgtgagctgcttccgacttgttcgggaactctctcttcatcctcttcgcgaccgcggccctccgctcccggccgcgcccgcccgccgccaggtaacccgctggactc

SEQ ID NO: 15983 - RNA, 7062 nt, Homo sapiens
  source 1..7062: mol_type = other RNA
gctgggattacaggcatgagccatcgcacctggccagtttttttttttttttttttttctaagtgcaatgggaagccactcaaagggctttaagcagggaagtgacattatctgattttcgttttataaagatccctgcggctgccgtcagtgattgtaggagggcaggagtggatgcaaggacagcagacattagtgcaggagttcaggtgaaagatgataatagcttgggcagagtggtagcagtggacatggagggaggtagacagatttaagatgtctcggagacagctgatggaatttgctgataactggaatgggagtgacaatgacaaataaaggaacctagaataagccccagaattttgcttaagcaactgagagttcagccatggcagatctgttaagcacaaaagttaaacacaaatacaaattcatactgcattggactcttttaagcagtgtcttatagaaaaaacattttatctagggaaaaatgcaacaacaaaaaccactgaaaacaaaagcctatgaataaaagcagacccgttttagactggatgcacaaaacaaaaacacacaggattcttgtggtggcgatgggagtaagtgaagacgtaacaggttgcaagttattttaaggactaagacccaatgttcagaaaccaaatcttgttcttccagtgtggatgcttagtcaaagactgtaaattgtcttcaagctgagagagaccatgaagagagaggagtggccacctaactaaccttcccagtttttgggagccaaacctagaccagaatgtaggtctaagtgactcccaatccagagctgtctccattaggccaggctctcaccccagctccaaaccaacttctaaaaacttgtccaagagtcctcctcttctttagaattggtaatcttggcaattaaattcagcgtagaaacactctcctgaacataatcagcatgctggttcttccttttctgttgccttgctcttcctaacagctcctcctttcgtctttgcaggctgcttctctgtcacaggaactcagggctcagtgctgtacttcatctccaaagtgtccctaaagcgcccatctgatcccatggctaactactccccaaattttctcctggactgaccttactgaatttagatttgtacatccaatacctgcttaacatatccactttgatgctcagtgggcacctcacacttgatctgtcaaacactgaatttctgtctctgttatgcacatacccaaactttccccaccatgtatttccccatctcaataaactgcaatagctcaagccaaaagcctaagattcagacctgaattctttcctttcctctctctcaaatgcaattcaacaattttcttaccttttattttttgttttggaatgaaggcacatataactgagctagtaataatgcttgattcataatacaccaccgatgttccatgcataactctcttattcatttgtccatgcatttattttgtttttgaatttttttaaaggggggcaaggtctacgttgcccaggttggaatatagtagctattcacaggtgaaatcatagcacactatagccttgaactggcctcaaggatcttcctatctcagactcccaagtagctgggactataagcacgcaccactacacccagctcatgtacttacttttaatgacaaatgaaccaccccaaaacccaccacctaacccagggactaaaacattaccagtgacttactcatagatttgctcctcctctacctctccagaggtaaccactatcttgaactttattactttttaaaagttttgtcacatatgtcaatgcctaaacagctgttcagttttagttgttcttgacttttataagaaaagtatcatgtcacatatagttttctcagaattgctttttcattctgagttattgtgctgcaagtagctggtattcattcattttgctgccatgtaataatcacccattctgtgaacacattacaccttcctaaaaatagacattttaatttattccagaacattcttatatgtgtgatctgggggacctgtgcaagcatttctcaagtatatactgaaaagtgaaattgctgacccatgggtatactttttttttttttttaaggtatgatcttactctgtcacccaaggtaagagtgcagtggcacaatcatgattcactgcagcctcaacctcctgggcttaagcaatccttccacctcagcttcccaagtagctgggaccacaggcatgcaccaccatgcccagctaattcaaaaaaatctttttgtgcagatgtggtctccctatgttgctcaagctggtcttgaactcttgggctcaagtgatcctcctaccttggcctcccaaagccaagaggcatgagccactgggcctggcccaacttttctagtgaatggtttttcacagtggatataccaattgatacccccatcagcaatatgtgagtgatcctaatgactaaaaccctctccaaaacttgactttgtgtttcttcattttcaccaatcgaatgaatttgaacatgtcattgtcatcttgatttacgttttcctgattgagagatgaaaacctcttaatgtttattggcccacatgcacttctaattgtgtggaaggcctggttcagtcttttgcctgtttttctgtgacactgtccttttttgttggtttgtagaatttctgcatacattcttgatactaagctattactagttataaatgttgcagatattgcctcacagtttgtagtttagctttagttttttttttagagacaaggtctccctatgttgcccaagttggacttgaacccctgggctcaagcaatcctcccacctcatcctcccaagttcatggacacagtgtgtgtgtgtgtgtgtgtgtgtgtgtgtgtgtaaatggagtttccctatttttcccaggcccgtctcaaactcctgggctcaagcagctcaagtaatccttctgcctctgcctcccaaagtgctgggattacaggcatgagccacaatgcctaactactgatgcacgatttctaaattaagaatttataatataccataacttatattcttttatggttatcttttatggtttttttttttcctgcttccagtttaagaagttcttcctaaagggagtaggatcaggaagataatcacattttctaaatatgtttcaatcacattttaatctataattccacatatagtttctacatcaagtcgtcatcctgttgcattaattttaaagagcatgcttctagtgtataaggttgaaaagcattcttccccttatagattactaaagatttattattaatgggtatactgattttctttagtcttactttttatttatcctttttaagtcatcaacaaactttttctgagtatttgattacctttctttcaaaccgtacagtatctcctggatttgtttctctttttatttaggtactttctccaaaagtgattttagtttgtacggaaaatcttctgaagctttgatggtacatattcttattaatgccctcacattagaataactattttcagaacataaaattgtaggttcaaagtttttttcaggttcaatttcacattcttgagctaggcatggtactgatggttttcaccataacatacaccaatgtccttttgtctgtgggctcccatccagcctggtggctgaagtcatctacaggtaagattgaccaaacctctgaacaggactgaaaaaaatgttatcttcagaaaaccagccctcttgtacactgctgctgtgaatacaaattgattaacttttctggatggcaatctagcaatgcagatcaaacatttaaaaatacatatatatctcgacacaattttatctccaggcatccacatgaaagaactccacaatgttcagaagtgtacagataaggatactcgtcacagcattataatatgaaaaataaactgaaaaccacctcatctccaaacacaattaaattatgttaaaattctataaacagggattaggatgtgtaggtttacccaagggaaaatatatttaatgtttaggtttaaaaagcaaaaaaaaagcctactttttgtttcaaaaatatgcatatgtaagtagaaaatatctgaaagctgaaaggctactatccaaaaatattaacagcagctttctctaaacagaaactaaagcagtttctcttttctttttgcttttctatacttattacatgtctaccacaaacctctttgttataatttctccagttgagtcagttttacaatttggaatgcagagatcaagtggttctataatcagcatatacttcgcacgtaccattcattcaatccacacccctttaaacccctttgacacacgtcaaactcatttacatctatgtccctccaatgacaatatagtggtcaacacatataaaacatgaatacactatatcaagacactcaggaatacatctctgggataaaatctgactgccttctattatattttaatgaataaccaaaataaagggattctttcagttacagagagcagaataattaaaatagtaactttcaaactttgtagcagcagaagtatttcttcaaataaaatcttttttgaaacccaatatagaaaacagataaaaataaagccattctagaggtgggggccttggaaagtgagtactatccactcagacttctttcttgcctctcacaaggaaggaagctactgtgtagtttgaaaattactatttaatacattctgctaaccctaaatgccatgtcagagctagaagagaaaatgtacacacattcaatctaacatttatttatttcaggttttttttttttttggcaactataaattacattcactagtacacctggaattcttcatagtgtgttcaactaaagaataagcaaacacagcatagatcagtttaaaagaaatcatggtacttcttagagcaatttgcaaaaggggaaaaaagtcttaggctcactccttggaaataaatatcaagtaaccataaaaatattcagccatttttcagttattcggggagttcaggcatggtcccacgcagagcatcagagttcctctttgaaataacccagctttgccaatgacatctcttttctcaactgcataacctcccaaaacatctgatcaacatcctgctgtttcacgagtccctgctgaatgtatcgaatgtatgtaaaaaagttacatacagaagtgatcctgtatctgcaaaaaggagaaatataataatagttgcttgagtcccctaatttaattctgtgtttacaggacttactctggccagtgagagcacatttttttggtcctccgcattcaactgcagaagctttcacaaaccggataggttgtaatcccactggttcaatgcttagagtattgttttccacagcctccagaacagctgaagccaactcactttttgagaatgttaaacatggaaagatatcttcctggtagattttgtctaagaaaggacacgtcctgtccattgtgggctcatccttccacaatcggaattcattatacaaggataagtcagcctctttgcagtcttttacaattggctgtatcacactgaggtcctgatgactgccactcatagcactgcttgtgcttttatttcttgtatgcccctttttaaaaggtgtctttccacctggcaaaggctcctgcgtaggtgatgttggagaactggacaatacaagtgtcttcaatgcagctacttcagcttgaagtacatcaatttttccttgtgcttcttttagctgtttttctgctgttgcctgcttgatatttgcttctctcaccattttatgagcttcctcaaatagactagctgtgagttcttccaattcctgtccaagttgatctcgcacttttgaaagcctctcacattcttcatcttttaacttcagttccctctgagcttttgcgagttcttcttttaatcgttcatagcccttttctctaacttccaaaacagatgggcttcgtaaacgagacagactatcagtactcaacccaaaaatatcatcactgccatcgcaagcctctgttatagtagcaccctgtaaaaactctctctctgcattatagttgtcctttcttgtagttaatttagttaatccagctgtgactccagaggtagagcaaggggctgggtctgtaacatgaaagctgatactagatatttccgcacaatttaaacgtctgggggatgaatacacgggttgtgtaggaagttcagaaacatctaatgcatttgcctggataggtacagaggataaagctgaagggtgtggccggtagatgacacttggtgaggtagtctgctcttgagttcctgattcatacacaccaagaaggtccggagaagtaggtgaagcaaggtttacttcatggaagccttccaagggatcattagccatagcaaaagcctcatcataagataaccctttcatcttttttaatcccataacaaccggcaactcttcacatgctgcgacttccacccagcatcatcacttctggagccagtaagctcgcgcttcctgggcggtcggggcgagttgtcaacgctgggagggcagagccatgcaatcccacccgtgcagttcgtctcaactcccccgaacacaagtctggcggcacggagctgcctacttgggcgcgactccgggcgcctgcccggaatttcccaccaggtttcaccgaaacctcccgagggtgacctctacgcctcagcacggtgcctcgcgcgtagtttcctaagactgggacacgaaaccaccccaggtccacagccctgccgcgcggcgtccggtgttgtgagctgcttccgacttgttcgggaactctctcttcatcctcttcgcgaccgcggccctccgctcccggccgcgcccgcccgccgccaggtaacccgctggactcgggctccct

SEQ ID NO: 15984 - RNA, 6677 nt, Homo sapiens
  source 1..6677: mol_type = other RNA
gctgggattacaggcatgagccatcgcacctggccagtttttttttttttttttttttctaagtgcaatgggaagccactcaaagggctttaagcagggaagtgacattatctgattttcgttttataaagatccctgcggctgccgtcagtgattgtaggagggcaggagtggatgcaaggacagcagacattagtgcaggagttcaggtgaaagatgataatagcttgggcagagtggtagcagtggacatggagggaggtagacagatttaagatgtctcggagacagctgatggaatttgctgataactggaatgggagtgacaatgacaaataaaggaacctagaataagccccagaattttgcttaagcaactgagagttcagccatggcagatctgttaagcacaaaagttaaacacaaatacaaattcatactgcattggactcttttaagcagtgtcttatagaaaaaacattttatctagggaaaaatgcaacaacaaaaaccactgaaaacaaaagcctatgaataaaagcagacccgttttagactggatgcacaaaacaaaaacacacaggattcttgtggtggcgatgggagtaagtgaagacgtaacaggttgcaagttattttaaggactaagacccaatgttcagaaaccaaatcttgttcttccagtgtggatgcttagtcaaagactgtaaattgtcttcaagctgagagagaccatgaagagagaggagtggccacctaactaaccttcccagtttttgggagccaaacctagaccagaatgtaggtctaagtgactcccaatccagagctgtctccattaggccaggctctcaccccagctccaaaccaacttctaaaaacttgtccaagagtcctcctcttctttagaattggtaatcttggcaattaaattcagcgtagaaacactctcctgaacataatcagcatgctggttcttccttttctgttgccttgctcttcctaacagctcctcctttcgtctttgcaggctgcttctctgtcacaggaactcagggctcagtgctgtacttcatctccaaagtgtccctaaagcgcccatctgatcccatggctaactactccccaaattttctcctggactgaccttactgaatttagatttgtacatccaatacctgcttaacatatccactttgatgctcagtgggcacctcacacttgatctgtcaaacactgaatttctgtctctgttatgcacatacccaaactttccccaccatgtatttccccatctcaataaactgcaatagctcaagccaaaagcctaagattcagacctgaattctttcctttcctctctctcaaatgcaattcaacaattttcttaccttttattttttgttttggaatgaaggcacatataactgagctagtaataatgcttgattcataatacaccaccgatgttccatgcataactctcttattcatttgtccatgcatttattttgtttttgaatttttttaaaggggggcaaggtctacgttgcccaggttggaatatagtagctattcacaggtgaaatcatagcacactatagccttgaactggcctcaaggatcttcctatctcagactcccaagtagctgggactataagcacgcaccactacacccagctcatgtacttacttttaatgacaaatgaaccaccccaaaacccaccacctaacccagggactaaaacattaccagtgacttactcatagatttgctcctcctctacctctccagaggtaaccactatcttgaactttattactttttaaaagttttgtcacatatgtcaatgcctaaacagctgttcagttttagttgttcttgacttttataagaaaagtatcatgtcacatatagttttctcagaattgctttttcattctgagttattgtgctgcaagtagctggtattcattcattttgctgccatgtaataatcacccattctgtgaacacattacaccttcctaaaaatagacattttaatttattccagaacattcttatatgtgtgatctgggggacctgtgcaagcatttctcaagtatatactgaaaagtgaaattgctgacccatgggtatactttttttttttttttaaggtatgatcttactctgtcacccaaggtaagagtgcagtggcacaatcatgattcactgcagcctcaacctcctgggcttaagcaatccttccacctcagcttcccaagtagctgggaccacaggcatgcaccaccatgcccagctaattcaaaaaaatctttttgtgcagatgtggtctccctatgttgctcaagctggtcttgaactcttgggctcaagtgatcctcctaccttggcctcccaaagccaagaggcatgagccactgggcctggcccaacttttctagtgaatggtttttcacagtggatataccaattgatacccccatcagcaatatgtgagtgatcctaatgactaaaaccctctccaaaacttgactttgtgtttcttcattttcaccaatcgaatgaatttgaacatgtcattgtcatcttgatttacgttttcctgattgagagatgaaaacctcttaatgtttattggcccacatgcacttctaattgtgtggaaggcctggttcagtcttttgcctgtttttctgtgacactgtccttttttgttggtttgtagaatttctgcatacattcttgatactaagctattactagttataaatgttgcagatattgcctcacagtttgtagtttagctttagttttttttttagagacaaggtctccctatgttgcccaagttggacttgaacccctgggctcaagcaatcctcccacctcatcctcccaagttcatggacacagtgtgtgtgtgtgtgtgtgtgtgtgtgtgtgtgtaaatggagtttccctatttttcccaggcccgtctcaaactcctgggctcaagcagctcaagtaatccttctgcctctgcctcccaaagtgctgggattacaggcatgagccacaatgcctaactactgatgcacgatttctaaattaagaatttataatataccataacttatattcttttatggttatcttttatggtttttttttttcctgcttccagtttaagaagttcttcctaaagggagtaggatcaggaagataatcacattttctaaatatgtttcaatcacattttaatctataattccacatatagtttctacatcaagtcgtcatcctgttgcattaattttaaagagcatgcttctagtgtataaggttgaaaagcattcttccccttatagattactaaagatttattattaatgggtatactgattttctttagtcttactttttatttatcctttttaagtcatcaacaaactttttctgagtatttgattacctttctttcaaaccgtacagtatctcctggatttgtttctctttttatttaggtactttctccaaaagtgattttagtttgtacggaaaatcttctgaagctttgatggtacatattcttattaatgccctcacattagaataactattttcagaacataaaattgtaggttcaaagtttttttcaggttcaatttcacattcttgagctaggcatggtactgatggttttcaccataacatacaccaatgtccttttgtctgtgggctcccatccagcctggtggctgaagtcatctacaggtaagattgaccaaacctctgaacaggactgaaaaaaatgttatcttcagaaaaccagccctcttgtacactgctgctgtgaatacaaattgattaacttttctggatggcaatctagcaatgcagatcaaacatttaaaaatacatatatatctcgacacaattttatctccaggcatccacatgaaagaactccacaatgttcagaagtgtacagataaggatactcgtcacagcattataatatgaaaaataaactgaaaaccacctcatctccaaacacaattaaattatgttaaaattctataaacagggattaggatgtgtaggtttacccaagggaaaatatatttaatgtttaggtttaaaaagcaaaaaaaaagcctactttttgtttcaaaaatatgcatatgtaagtagaaaatatctgaaagctgaaaggctactatccaaaaatattaacagcagctttctctaaacagaaactaaagcagtttctcttttctttttgcttttctatacttattacatgtctaccacaaacctctttgttataatttctccagttgagtcagttttacaatttggaatgcagagatcaagtggttctataatcagcatatacttcgcacgtaccattcattcaatccacacccctttaaacccctttgacacacgtcaaactcatttacatctatgtccctccaatgacaatatagtggtcaacacatataaaacatgaatacactatatcaagacactcaggaatacatctctgggataaaatctgactgccttctattatattttaatgaataaccaaaataaagggattctttcagttacagagagcagaataattaaaatagtaactttcaaactttgtagcagcagaagtatttcttcaaataaaatcttttttgaaacccaatatagaaaacagataaaaataaagccattctagaggtgggggccttggaaagtgagtactatccactcagacttctttcttgcctctcacaaggaaggaagctactgtgtagtttgaaaattactatttaatacattctgctaaccctaaatgccatgtcagagctagaagagaaaatgtacacacattcaatctaacatttatttatttcaggttttttttttttttggcaactataaattacattcactagtacacctggaattcttcatagtgtgttcaactaaagaataagcaaacacagcatagatcagtttaaaagaaatcatggtacttcttagagcaatttgcaaaaggggaaaaaagtcttaggctcactccttggaaataaatatcaagtaaccataaaaatattcagccatttttcagttattcggggagttcaggcatggtcccacgcagagcatcagagttcctctttgaaataacccagctttgccaatgacatctcttttctcaactgcataacctcccaaaacatctgatcaacatcctgctgtttcacgagtccctgctgaatgtatcgaatgtatgtaaaaaagttacatacagaagtgatcctgtatctgcaaaaaggagaaatataataatagttgcttgagtcccctaatttaattctgtgtttacaggacttactctggccagtgagagcacatttttttggtcctccgcattcaactgcagaagctttcacaaaccggataggttgtaatcccactggttcaatgcttagagtattgttttccacagcctccagaacagctgaagccaactcactttttgagaatgttaaacatggaaagatatcttcctggtagattttgtctaagaaaggacacgtcctgtccattgtgggctcatccttccacaatcggaattcattatacaaggataagtcagcctctttgcagtcttttacaattggctgtatcacactgaggtcctgatgactgccactcatagcactgcttgtgcttttatttcttgtatgcccctttttaaaaggtgtctttccacctggcaaaggctcctgcgtaggtgatgttggagaactggacaatacaagtgtcttcaatgcagctacttcagcttgaagtacatcaatttttccttgtgcttcttttagctgtttttctgctgttgcctgcttgatatttgcttctctcaccattttatgagcttcctcaaatagactagctgtgagttcttccaattcctgtccaagttgatctcgcacttttgaaagcctctcacattcttcatcttttaacttcagttccctctgagcttttgcgagttcttcttttaatcgttcatagcccttttctctaacttccaaaacagatgggcttcgtaaacgagacagactatcagtactcaacccaaaaatatcatcactgccatcgcaagcctctgttatagtagcaccctgtaaaaactctctctctgcattatagttgtcctttcttgtagttaatttagttaatccagctgtgactccagaggtagagcaaggggctgggtctgtaacatgaaagctgatactagatatttccgcacaatttaaacgtctgggggatgaatacacgggttgtgtaggaagttcagaaacatctaatgcatttgcctggataggtacagaggataaagctgaagggtgtggccggtagatgacacttggtgaggtagtctgctcttgagttcctgattcatacacaccaagaaggtccggagaagtaggtgaagcaaggtttacttcatggaagccttccaagggatcattagccatagcaaaagcctcatcataagataacctgaactcactgatcacatcttgtcacaaaaacggagacaatcaaacattatgtatattatgtggcaaataagaaatgaacatcactgccattaataaagcatt

SEQ ID NO: 15985 - RNA, 6745 nt, Homo sapiens
  source 1..6745: mol_type = other RNA
gctgggattacaggcatgagccatcgcacctggccagtttttttttttttttttttttctaagtgcaatgggaagccactcaaagggctttaagcagggaagtgacattatctgattttcgttttataaagatccctgcggctgccgtcagtgattgtaggagggcaggagtggatgcaaggacagcagacattagtgcaggagttcaggtgaaagatgataatagcttgggcagagtggtagcagtggacatggagggaggtagacagatttaagatgtctcggagacagctgatggaatttgctgataactggaatgggagtgacaatgacaaataaaggaacctagaataagccccagaattttgcttaagcaactgagagttcagccatggcagatctgttaagcacaaaagttaaacacaaatacaaattcatactgcattggactcttttaagcagtgtcttatagaaaaaacattttatctagggaaaaatgcaacaacaaaaaccactgaaaacaaaagcctatgaataaaagcagacccgttttagactggatgcacaaaacaaaaacacacaggattcttgtggtggcgatgggagtaagtgaagacgtaacaggttgcaagttattttaaggactaagacccaatgttcagaaaccaaatcttgttcttccagtgtggatgcttagtcaaagactgtaaattgtcttcaagctgagagagaccatgaagagagaggagtggccacctaactaaccttcccagtttttgggagccaaacctagaccagaatgtaggtctaagtgactcccaatccagagctgtctccattaggccaggctctcaccccagctccaaaccaacttctaaaaacttgtccaagagtcctcctcttctttagaattggtaatcttggcaattaaattcagcgtagaaacactctcctgaacataatcagcatgctggttcttccttttctgttgccttgctcttcctaacagctcctcctttcgtctttgcaggctgcttctctgtcacaggaactcagggctcagtgctgtacttcatctccaaagtgtccctaaagcgcccatctgatcccatggctaactactccccaaattttctcctggactgaccttactgaatttagatttgtacatccaatacctgcttaacatatccactttgatgctcagtgggcacctcacacttgatctgtcaaacactgaatttctgtctctgttatgcacatacccaaactttccccaccatgtatttccccatctcaataaactgcaatagctcaagccaaaagcctaagattcagacctgaattctttcctttcctctctctcaaatgcaattcaacaattttcttaccttttattttttgttttggaatgaaggcacatataactgagctagtaataatgcttgattcataatacaccaccgatgttccatgcataactctcttattcatttgtccatgcatttattttgtttttgaatttttttaaaggggggcaaggtctacgttgcccaggttggaatatagtagctattcacaggtgaaatcatagcacactatagccttgaactggcctcaaggatcttcctatctcagactcccaagtagctgggactataagcacgcaccactacacccagctcatgtacttacttttaatgacaaatgaaccaccccaaaacccaccacctaacccagggactaaaacattaccagtgacttactcatagatttgctcctcctctacctctccagaggtaaccactatcttgaactttattactttttaaaagttttgtcacatatgtcaatgcctaaacagctgttcagttttagttgttcttgacttttataagaaaagtatcatgtcacatatagttttctcagaattgctttttcattctgagttattgtgctgcaagtagctggtattcattcattttgctgccatgtaataatcacccattctgtgaacacattacaccttcctaaaaatagacattttaatttattccagaacattcttatatgtgtgatctgggggacctgtgcaagcatttctcaagtatatactgaaaagtgaaattgctgacccatgggtatactttttttttttttttaaggtatgatcttactctgtcacccaaggtaagagtgcagtggcacaatcatgattcactgcagcctcaacctcctgggcttaagcaatccttccacctcagcttcccaagtagctgggaccacaggcatgcaccaccatgcccagctaattcaaaaaaatctttttgtgcagatgtggtctccctatgttgctcaagctggtcttgaactcttgggctcaagtgatcctcctaccttggcctcccaaagccaagaggcatgagccactgggcctggcccaacttttctagtgaatggtttttcacagtggatataccaattgatacccccatcagcaatatgtgagtgatcctaatgactaaaaccctctccaaaacttgactttgtgtttcttcattttcaccaatcgaatgaatttgaacatgtcattgtcatcttgatttacgttttcctgattgagagatgaaaacctcttaatgtttattggcccacatgcacttctaattgtgtggaaggcctggttcagtcttttgcctgtttttctgtgacactgtccttttttgttggtttgtagaatttctgcatacattcttgatactaagctattactagttataaatgttgcagatattgcctcacagtttgtagtttagctttagttttttttttagagacaaggtctccctatgttgcccaagttggacttgaacccctgggctcaagcaatcctcccacctcatcctcccaagttcatggacacagtgtgtgtgtgtgtgtgtgtgtgtgtgtgtgtgtaaatggagtttccctatttttcccaggcccgtctcaaactcctgggctcaagcagctcaagtaatccttctgcctctgcctcccaaagtgctgggattacaggcatgagccacaatgcctaactactgatgcacgatttctaaattaagaatttataatataccataacttatattcttttatggttatcttttatggtttttttttttcctgcttccagtttaagaagttcttcctaaagggagtaggatcaggaagataatcacattttctaaatatgtttcaatcacattttaatctataattccacatatagtttctacatcaagtcgtcatcctgttgcattaattttaaagagcatgcttctagtgtataaggttgaaaagcattcttccccttatagattactaaagatttattattaatgggtatactgattttctttagtcttactttttatttatcctttttaagtcatcaacaaactttttctgagtatttgattacctttctttcaaaccgtacagtatctcctggatttgtttctctttttatttaggtactttctccaaaagtgattttagtttgtacggaaaatcttctgaagctttgatggtacatattcttattaatgccctcacattagaataactattttcagaacataaaattgtaggttcaaagtttttttcaggttcaatttcacattcttgagctaggcatggtactgatggttttcaccataacatacaccaatgtccttttgtctgtgggctcccatccagcctggtggctgaagtcatctacaggtaagattgaccaaacctctgaacaggactgaaaaaaatgttatcttcagaaaaccagccctcttgtacactgctgctgtgaatacaaattgattaacttttctggatggcaatctagcaatgcagatcaaacatttaaaaatacatatatatctcgacacaattttatctccaggcatccacatgaaagaactccacaatgttcagaagtgtacagataaggatactcgtcacagcattataatatgaaaaataaactgaaaaccacctcatctccaaacacaattaaattatgttaaaattctataaacagggattaggatgtgtaggtttacccaagggaaaatatatttaatgtttaggtttaaaaagcaaaaaaaaagcctactttttgtttcaaaaatatgcatatgtaagtagaaaatatctgaaagctgaaaggctactatccaaaaatattaacagcagctttctctaaacagaaactaaagcagtttctcttttctttttgcttttctatacttattacatgtctaccacaaacctctttgttataatttctccagttgagtcagttttacaatttggaatgcagagatcaagtggttctataatcagcatatacttcgcacgtaccattcattcaatccacacccctttaaacccctttgacacacgtcaaactcatttacatctatgtccctccaatgacaatatagtggtcaacacatataaaacatgaatacactatatcaagacactcaggaatacatctctgggataaaatctgactgccttctattatattttaatgaataaccaaaataaagggattctttcagttacagagagcagaataattaaaatagtaactttcaaactttgtagcagcagaagtatttcttcaaataaaatcttttttgaaacccaatatagaaaacagataaaaataaagccattctagaggtgggggccttggaaagtgagtactatccactcagacttctttcttgcctctcacaaggaaggaagctactgtgtagtttgaaaattactatttaatacattctgctaaccctaaatgccatgtcagagctagaagagaaaatgtacacacattcaatctaacatttatttatttcaggttttttttttttttggcaactataaattacattcactagtacacctggaattcttcatagtgtgttcaactaaagaataagcaaacacagcatagatcagtttaaaagaaatcatggtacttcttagagcaatttgcaaaaggggaaaaaagtcttaggctcactccttggaaataaatatcaagtaaccataaaaatattcagccatttttcagttattcggggagttcaggcatggtcccacgcagagcatcagagttcctctttgaaataacccagctttgccaatgacatctcttttctcaactgcataacctcccaaaacatctgatcaacatcctgctgtttcacgagtccctgctgaatgtatcgaatgtatgtaaaaaagttacatacagaagtgatcctgtatctgcaaaaaggagaaatataataatagttgcttgagtcccctaatttaattctgtgtttacaggacttactctggccagtgagagcacatttttttggtcctccgcattcaactgcagaagctttcacaaaccggataggttgtaatcccactggttcaatgcttagagtattgttttccacagcctccagaacagctgaagccaactcactttttgagaatgttaaacatggaaagatatcttcctggtagattttgtctaagaaaggacacgtcctgtccattgtgggctcatccttccacaatcggaattcattatacaaggataagtcagcctctttgcagtcttttacaattggctgtatcacactgaggtcctgatgactgccactcatagcactgcttgtgcttttatttcttgtatgcccctttttaaaaggtgtctttccacctggcaaaggctcctgcgtaggtgatgttggagaactggacaatacaagtgtcttcaatgcagctacttcagcttgaagtacatcaatttttccttgtgcttcttttagctgtttttctgctgttgcctgcttgatatttgcttctctcaccattttatgagcttcctcaaatagactagctgtgagttcttccaattcctgtccaagttgatctcgcacttttgaaagcctctcacattcttcatcttttaacttcagttccctctgagcttttgcgagttcttcttttaatcgttcatagcccttttctctaacttccaaaacagatgggcttcgtaaacgagacagactatcagtactcaacccaaaaatatcatcactgccatcgcaagcctctgttatagtagcaccctgtaaaaactctctctctgcattatagttgtcctttcttgtagttaatttagttaatccagctgtgactccagaggtagagcaaggggctgggtctgtaacatgaaagctgatactagatatttccgcacaatttaaacgtctgggggatgaatacacgggttgtgtaggaagttcagaaacatctaatgcatttgcctggataggtacagaggataaagctgaagggtgtggccggtagatgacacttggtgaggtagtctgctcttgagttcctgattcatacacaccaagaaggtccggagaagtaggtgaagcaaggtttacttcatggaagccttccaagggatcattagccatagcaaaagcctcatcataagataacctgaagaacccaccgcggccgctgccggcgctcaggggcgctcacagagccgcagagagcgcgtcccgaagcagcgagaaacggaggaggacggcgagccctttccgctacactccacggcggcgggctcactacgccggcagccgccgagggaacgcgggactgcgcctgc

SEQ ID NO: 15986 - RNA, 7042 nt, Homo sapiens
  source 1..7042: mol_type = other RNA
gctgggattacaggcatgagccatcgcacctggccagtttttttttttttttttttttctaagtgcaatgggaagccactcaaagggctttaagcagggaagtgacattatctgattttcgttttataaagatccctgcggctgccgtcagtgattgtaggagggcaggagtggatgcaaggacagcagacattagtgcaggagttcaggtgaaagatgataatagcttgggcagagtggtagcagtggacatggagggaggtagacagatttaagatgtctcggagacagctgatggaatttgctgataactggaatgggagtgacaatgacaaataaaggaacctagaataagccccagaattttgcttaagcaactgagagttcagccatggcagatctgttaagcacaaaagttaaacacaaatacaaattcatactgcattggactcttttaagcagtgtcttatagaaaaaacattttatctagggaaaaatgcaacaacaaaaaccactgaaaacaaaagcctatgaataaaagcagacccgttttagactggatgcacaaaacaaaaacacacaggattcttgtggtggcgatgggagtaagtgaagacgtaacaggttgcaagttattttaaggactaagacccaatgttcagaaaccaaatcttgttcttccagtgtggatgcttagtcaaagactgtaaattgtcttcaagctgagagagaccatgaagagagaggagtggccacctaactaaccttcccagtttttgggagccaaacctagaccagaatgtaggtctaagtgactcccaatccagagctgtctccattaggccaggctctcaccccagctccaaaccaacttctaaaaacttgtccaagagtcctcctcttctttagaattggtaatcttggcaattaaattcagcgtagaaacactctcctgaacataatcagcatgctggttcttccttttctgttgccttgctcttcctaacagctcctcctttcgtctttgcaggctgcttctctgtcacaggaactcagggctcagtgctgtacttcatctccaaagtgtccctaaagcgcccatctgatcccatggctaactactccccaaattttctcctggactgaccttactgaatttagatttgtacatccaatacctgcttaacatatccactttgatgctcagtgggcacctcacacttgatctgtcaaacactgaatttctgtctctgttatgcacatacccaaactttccccaccatgtatttccccatctcaataaactgcaatagctcaagccaaaagcctaagattcagacctgaattctttcctttcctctctctcaaatgcaattcaacaattttcttaccttttattttttgttttggaatgaaggcacatataactgagctagtaataatgcttgattcataatacaccaccgatgttccatgcataactctcttattcatttgtccatgcatttattttgtttttgaatttttttaaaggggggcaaggtctacgttgcccaggttggaatatagtagctattcacaggtgaaatcatagcacactatagccttgaactggcctcaaggatcttcctatctcagactcccaagtagctgggactataagcacgcaccactacacccagctcatgtacttacttttaatgacaaatgaaccaccccaaaacccaccacctaacccagggactaaaacattaccagtgacttactcatagatttgctcctcctctacctctccagaggtaaccactatcttgaactttattactttttaaaagttttgtcacatatgtcaatgcctaaacagctgttcagttttagttgttcttgacttttataagaaaagtatcatgtcacatatagttttctcagaattgctttttcattctgagttattgtgctgcaagtagctggtattcattcattttgctgccatgtaataatcacccattctgtgaacacattacaccttcctaaaaatagacattttaatttattccagaacattcttatatgtgtgatctgggggacctgtgcaagcatttctcaagtatatactgaaaagtgaaattgctgacccatgggtatactttttttttttttttaaggtatgatcttactctgtcacccaaggtaagagtgcagtggcacaatcatgattcactgcagcctcaacctcctgggcttaagcaatccttccacctcagcttcccaagtagctgggaccacaggcatgcaccaccatgcccagctaattcaaaaaaatctttttgtgcagatgtggtctccctatgttgctcaagctggtcttgaactcttgggctcaagtgatcctcctaccttggcctcccaaagccaagaggcatgagccactgggcctggcccaacttttctagtgaatggtttttcacagtggatataccaattgatacccccatcagcaatatgtgagtgatcctaatgactaaaaccctctccaaaacttgactttgtgtttcttcattttcaccaatcgaatgaatttgaacatgtcattgtcatcttgatttacgttttcctgattgagagatgaaaacctcttaatgtttattggcccacatgcacttctaattgtgtggaaggcctggttcagtcttttgcctgtttttctgtgacactgtccttttttgttggtttgtagaatttctgcatacattcttgatactaagctattactagttataaatgttgcagatattgcctcacagtttgtagtttagctttagttttttttttagagacaaggtctccctatgttgcccaagttggacttgaacccctgggctcaagcaatcctcccacctcatcctcccaagttcatggacacagtgtgtgtgtgtgtgtgtgtgtgtgtgtgtgtgtaaatggagtttccctatttttcccaggcccgtctcaaactcctgggctcaagcagctcaagtaatccttctgcctctgcctcccaaagtgctgggattacaggcatgagccacaatgcctaactactgatgcacgatttctaaattaagaatttataatataccataacttatattcttttatggttatcttttatggtttttttttttcctgcttccagtttaagaagttcttcctaaagggagtaggatcaggaagataatcacattttctaaatatgtttcaatcacattttaatctataattccacatatagtttctacatcaagtcgtcatcctgttgcattaattttaaagagcatgcttctagtgtataaggttgaaaagcattcttccccttatagattactaaagatttattattaatgggtatactgattttctttagtcttactttttatttatcctttttaagtcatcaacaaactttttctgagtatttgattacctttctttcaaaccgtacagtatctcctggatttgtttctctttttatttaggtactttctccaaaagtgattttagtttgtacggaaaatcttctgaagctttgatggtacatattcttattaatgccctcacattagaataactattttcagaacataaaattgtaggttcaaagtttttttcaggttcaatttcacattcttgagctaggcatggtactgatggttttcaccataacatacaccaatgtccttttgtctgtgggctcccatccagcctggtggctgaagtcatctacaggtaagattgaccaaacctctgaacaggactgaaaaaaatgttatcttcagaaaaccagccctcttgtacactgctgctgtgaatacaaattgattaacttttctggatggcaatctagcaatgcagatcaaacatttaaaaatacatatatatctcgacacaattttatctccaggcatccacatgaaagaactccacaatgttcagaagtgtacagataaggatactcgtcacagcattataatatgaaaaataaactgaaaaccacctcatctccaaacacaattaaattatgttaaaattctataaacagggattaggatgtgtaggtttacccaagggaaaatatatttaatgtttaggtttaaaaagcaaaaaaaaagcctactttttgtttcaaaaatatgcatatgtaagtagaaaatatctgaaagctgaaaggctactatccaaaaatattaacagcagctttctctaaacagaaactaaagcagtttctcttttctttttgcttttctatacttattacatgtctaccacaaacctctttgttataatttctccagttgagtcagttttacaatttggaatgcagagatcaagtggttctataatcagcatatacttcgcacgtaccattcattcaatccacacccctttaaacccctttgacacacgtcaaactcatttacatctatgtccctccaatgacaatatagtggtcaacacatataaaacatgaatacactatatcaagacactcaggaatacatctctgggataaaatctgactgccttctattatattttaatgaataaccaaaataaagggattctttcagttacagagagcagaataattaaaatagtaactttcaaactttgtagcagcagaagtatttcttcaaataaaatcttttttgaaacccaatatagaaaacagataaaaataaagccattctagaggtgggggccttggaaagtgagtactatccactcagacttctttcttgcctctcacaaggaaggaagctactgtgtagtttgaaaattactatttaatacattctgctaaccctaaatgccatgtcagagctagaagagaaaatgtacacacattcaatctaacatttatttatttcaggttttttttttttttggcaactataaattacattcactagtacacctggaattcttcatagtgtgttcaactaaagaataagcaaacacagcatagatcagtttaaaagaaatcatggtacttcttagagcaatttgcaaaaggggaaaaaagtcttaggctcactccttggaaataaatatcaagtaaccataaaaatattcagccatttttcagttattcggggagttcaggcatggtcccacgcagagcatcagagttcctctttgaaataacccagctttgccaatgacatctcttttctcaactgcataacctcccaaaacatctgatcaacatcctgctgtttcacgagtccctgctgaatgtatcgaatgtatgtaaaaaagttacatacagaagtgatcctgtatctgcaaaaaggagaaatataataatagttgcttgagtcccctaatttaattctgtgtttacaggacttactctggccagtgagagcacatttttttggtcctccgcattcaactgcagaagctttcacaaaccggataggttgtaatcccactggttcaatgcttagagtattgttttccacagcctccagaacagctgaagccaactcactttttgagaatgttaaacatggaaagatatcttcctggtagattttgtctaagaaaggacacgtcctgtccattgtgggctcatccttccacaatcggaattcattatacaaggataagtcagcctctttgcagtcttttacaattggctgtatcacactgaggtcctgatgactgccactcatagcactgcttgtgcttttatttcttgtatgcccctttttaaaaggtgtctttccacctggcaaaggctcctgcgtaggtgatgttggagaactggacaatacaagtgtcttcaatgcagctacttcagcttgaagtacatcaatttttccttgtgcttcttttagctgtttttctgctgttgcctgcttgatatttgcttctctcaccattttatgagcttcctcaaatagactagctgtgagttcttccaattcctgtccaagttgatctcgcacttttgaaagcctctcacattcttcatcttttaacttcagttccctctgagcttttgcgagttcttcttttaatcgttcatagcccttttctctaacttccaaaacagatgggcttcgtaaacgagacagactatcagtactcaacccaaaaatatcatcactgccatcgcaagcctctgttatagtagcaccctgtaaaaactctctctctgcattatagttgtcctttcttgtagttaatttagttaatccagctgtgactccagaggtagagcaaggggctgggtctgtaacatgaaagctgatactagatatttccgcacaatttaaacgtctgggggatgaatacacgggttgtgtaggaagttcagaaacatctaatgcatttgcctggataggtacagaggataaagctgaagggtgtggccggtagatgacacttggtgaggtagtctgctcttgagttcctgattcatacacaccaagaaggtccggagaagtaggtgaagcaaggtttacttcatggaagccttccaagggatcattagccatagcaaaagcctcatcataagataacctgagactccgcggccatatacaccttacgacgtgtgtgtgtgtggcgggagatgggaggggaggaatcctgtagaacccagatcccatcattccagcaactgccagagcgttcgagaatgtcatgtctgtacctgtcttctctcatcttttgtgccaactgttttatcaaacttctaccccactttaggtcttccaggtaggaaaaatacagaaagagccaagatcccaaaaatcaaaaaaaaataataataatagaggtagtcatagtatgtgtctctatgtttagcaaaagagaaacgtgcatttgtgtgatacacttattgaataggaccatcattctgggtattaatctcatctattagaggcagtaaagaaaagtagactatatgtatggttgttggagtcagaattactgggcttgagcctgccacctgctagctgagtgaccttaggcaaatgaatctctc

SEQ ID NO: 15987 - RNA, 6268 nt, Homo sapiens
  source 1..6268: mol_type = other RNA
gctgggattacaggcatgagccatcgcacctggccagtttttttttttttttttttttctaagtgcaatgggaagccactcaaagggctttaagcagggaagtgacattatctgattttcgttttataaagatccctgcggctgccgtcagtgattgtaggagggcaggagtggatgcaaggacagcagacattagtgcaggagttcaggtgaaagatgataatagcttgggcagagtggtagcagtggacatggagggaggtagacagatttaagatgtctcggagacagctgatggaatttgctgataactggaatgggagtgacaatgacaaataaaggaacctagaataagccccagaattttgcttaagcaactgagagttcagccatggcagatctgttaagcacaaaagttaaacacaaatacaaattcatactgcattggactcttttaagcagtgtcttatagaaaaaacattttatctagggaaaaatgcaacaacaaaaaccactgaaaacaaaagcctatgaataaaagcagacccgttttagactggatgcacaaaacaaaaacacacaggattcttgtggtggcgatgggagtaagtgaagacgtaacaggttgcaagttattttaaggactaagacccaatgttcagaaaccaaatcttgttcttccagtgtggatgcttagtcaaagactgtaaattgtcttcaagctgagagagaccatgaagagagaggagtggccacctaactaaccttcccagtttttgggagccaaacctagaccagaatgtaggtctaagtgactcccaatccagagctgtctccattaggccaggctctcaccccagctccaaaccaacttctaaaaacttgtccaagagtcctcctcttctttagaattggtaatcttggcaattaaattcagcgtagaaacactctcctgaacataatcagcatgctggttcttccttttctgttgccttgctcttcctaacagctcctcctttcgtctttgcaggctgcttctctgtcacaggaactcagggctcagtgctgtacttcatctccaaagtgtccctaaagcgcccatctgatcccatggctaactactccccaaattttctcctggactgaccttactgaatttagatttgtacatccaatacctgcttaacatatccactttgatgctcagtgggcacctcacacttgatctgtcaaacactgaatttctgtctctgttatgcacatacccaaactttccccaccatgtatttccccatctcaataaactgcaatagctcaagccaaaagcctaagattcagacctgaattctttcctttcctctctctcaaatgcaattcaacaattttcttaccttttattttttgttttggaatgaaggcacatataactgagctagtaataatgcttgattcataatacaccaccgatgttccatgcataactctcttattcatttgtccatgcatttattttgtttttgaatttttttaaaggggggcaaggtctacgttgcccaggttggaatatagtagctattcacaggtgaaatcatagcacactatagccttgaactggcctcaaggatcttcctatctcagactcccaagtagctgggactataagcacgcaccactacacccagctcatgtacttacttttaatgacaaatgaaccaccccaaaacccaccacctaacccagggactaaaacattaccagtgacttactcatagatttgctcctcctctacctctccagaggtaaccactatcttgaactttattactttttaaaagttttgtcacatatgtcaatgcctaaacagctgttcagttttagttgttcttgacttttataagaaaagtatcatgtcacatatagttttctcagaattgctttttcattctgagttattgtgctgcaagtagctggtattcattcattttgctgccatgtaataatcacccattctgtgaacacattacaccttcctaaaaatagacattttaatttattccagaacattcttatatgtgtgatctgggggacctgtgcaagcatttctcaagtatatactgaaaagtgaaattgctgacccatgggtatactttttttttttttttaaggtatgatcttactctgtcacccaaggtaagagtgcagtggcacaatcatgattcactgcagcctcaacctcctgggcttaagcaatccttccacctcagcttcccaagtagctgggaccacaggcatgcaccaccatgcccagctaattcaaaaaaatctttttgtgcagatgtggtctccctatgttgctcaagctggtcttgaactcttgggctcaagtgatcctcctaccttggcctcccaaagccaagaggcatgagccactgggcctggcccaacttttctagtgaatggtttttcacagtggatataccaattgatacccccatcagcaatatgtgagtgatcctaatgactaaaaccctctccaaaacttgactttgtgtttcttcattttcaccaatcgaatgaatttgaacatgtcattgtcatcttgatttacgttttcctgattgagagatgaaaacctcttaatgtttattggcccacatgcacttctaattgtgtggaaggcctggttcagtcttttgcctgtttttctgtgacactgtccttttttgttggtttgtagaatttctgcatacattcttgatactaagctattactagttataaatgttgcagatattgcctcacagtttgtagtttagctttagttttttttttagagacaaggtctccctatgttgcccaagttggacttgaacccctgggctcaagcaatcctcccacctcatcctcccaagttcatggacacagtgtgtgtgtgtgtgtgtgtgtgtgtgtgtgtgtaaatggagtttccctatttttcccaggcccgtctcaaactcctgggctcaagcagctcaagtaatccttctgcctctgcctcccaaagtgctgggattacaggcatgagccacaatgcctaactactgatgcacgatttctaaattaagaatttataatataccataacttatattcttttatggttatcttttatggtttttttttttcctgcttccagtttaagaagttcttcctaaagggagtaggatcaggaagataatcacattttctaaatatgtttcaatcacattttaatctataattccacatatagtttctacatcaagtcgtcatcctgttgcattaattttaaagagcatgcttctagtgtataaggttgaaaagcattcttccccttatagattactaaagatttattattaatgggtatactgattttctttagtcttactttttatttatcctttttaagtcatcaacaaactttttctgagtatttgattacctttctttcaaaccgtacagtatctcctggatttgtttctctttttatttaggtactttctccaaaagtgattttagtttgtacggaaaatcttctgaagctttgatggtacatattcttattaatgccctcacattagaataactattttcagaacataaaattgtaggttcaaagtttttttcaggttcaatttcacattcttgagctaggcatggtactgatggttttcaccataacatacaccaatgtccttttgtctgtgggctcccatccagcctggtggctgaagtcatctacaggtaagattgaccaaacctctgaacaggactgaaaaaaatgttatcttcagaaaaccagccctcttgtacactgctgctgtgaatacaaattgattaacttttctggatggcaatctagcaatgcagatcaaacatttaaaaatacatatatatctcgacacaattttatctccaggcatccacatgaaagaactccacaatgttcagaagtgtacagataaggatactcgtcacagcattataatatgaaaaataaactgaaaaccacctcatctccaaacacaattaaattatgttaaaattctataaacagggattaggatgtgtaggtttacccaagggaaaatatatttaatgtttaggtttaaaaagcaaaaaaaaagcctactttttgtttcaaaaatatgcatatgtaagtagaaaatatctgaaagctgaaaggctactatccaaaaatattaacagcagctttctctaaacagaaactaaagcagtttctcttttctttttgcttttctatacttattacatgtctaccacaaacctctttgttataatttctccagttgagtcagttttacaatttggaatgcagagatcaagtggttctataatcagcatatacttcgcacgtaccattcattcaatccacacccctttaaacccctttgacacacgtcaaactcatttacatctatgtccctccaatgacaatatagtggtcaacacatataaaacatgaatacactatatcaagacactcaggaatacatctctgggataaaatctgactgccttctattatattttaatgaataaccaaaataaagggattctttcagttacagagagcagaataattaaaatagtaactttcaaactttgtagcagcagaagtatttcttcaaataaaatcttttttgaaacccaatatagaaaacagataaaaataaagccattctagaggtgggggccttggaaagtgagtactatccactcagacttctttcttgcctctcacaaggaaggaagctactgtgtagtttgaaaattactatttaatacattctgctaaccctaaatgccatgtcagagctagaagagaaaatgtacacacattcaatctaacatttatttatttcaggttttttttttttttggcaactataaattacattcactagtacacctggaattcttcatagtgtgttcaactaaagaataagcaaacacagcatagatcagtttaaaagaaatcatggtacttcttagagcaatttgcaaaaggggaaaaaagtcttaggctcactccttggaaataaatatcaagtaaccataaaaatattcagccatttttcagttattcggggagttcaggcatggtcccacgcagagcatcagagttcctctttgaaataacccagctttgccaatgacatctcttttctcaactgcataacctcccaaaacatctgatcaacatcctgctgtttcacgagtccctgctgaatgtatcgaatgtatgtaaaaaagttacatacagaagtgatcctgtatctgcaaaaaggagaaatataataatagttgcttgagtcccctaatttaattctgtgtttacaggacttactctggccagtgagagcacatttttttggtcctccgcattcaactgcagaagctttcacaaaccggataggttgtaatcccactggttcaatgcttagagtattgttttccacagcctccagaacagctgaagccaactcactttttgagaatgttaaacatggaaagatatcttcctggtagattttgtctaagaaaggacacgtcctgtccattgtgggctcatccttccacaatcggaattcattatacaaggataagtcagcctctttgcagtcttttacaattggctgtatcacactgaggtcctgatgactgccactcatagcactgcttgtgcttttatttcttgtatgcccctttttaaaaggtgtctttccacctggcaaaggctcctgcgtaggtgatgttggagaactggacaatacaagtgtcttcaatgcagctacttcagcttgaagtacatcaatttttccttgtgcttcttttagctgtttttctgctgttgcctgcttgatatttgcttctctcaccattttatgagcttcctcaaatagactagctgtgagttcttccaattcctgtccaagttgatctcgcacttttgaaagcctctcacattcttcatcttttaacttcagttcctggaaaatcgggtcactcccatccgaatattgcgcttttcagaccggcttaagaaacggcgcaccacgagactatatcccacacctggctcagagggtcctacgcccacggaatctcgctgattgctagcacagcagtctgagatcaaactgcaaggcggcaacgaggctgggggagggacgcccgccattgcccaggcttgcttaggtaaacaaagcagccgggaagc

SEQ ID NO: 15988 - RNA, 6183 nt, Homo sapiens
  source 1..6183: mol_type = other RNA
gctgggattacaggcatgagccatcgcacctggccagtttttttttttttttttttttctaagtgcaatgggaagccactcaaagggctttaagcagggaagtgacattatctgattttcgttttataaagatccctgcggctgccgtcagtgattgtaggagggcaggagtggatgcaaggacagcagacattagtgcaggagttcaggtgaaagatgataatagcttgggcagagtggtagcagtggacatggagggaggtagacagatttaagatgtctcggagacagctgatggaatttgctgataactggaatgggagtgacaatgacaaataaaggaacctagaataagccccagaattttgcttaagcaactgagagttcagccatggcagatctgttaagcacaaaagttaaacacaaatacaaattcatactgcattggactcttttaagcagtgtcttatagaaaaaacattttatctagggaaaaatgcaacaacaaaaaccactgaaaacaaaagcctatgaataaaagcagacccgttttagactggatgcacaaaacaaaaacacacaggattcttgtggtggcgatgggagtaagtgaagacgtaacaggttgcaagttattttaaggactaagacccaatgttcagaaaccaaatcttgttcttccagtgtggatgcttagtcaaagactgtaaattgtcttcaagctgagagagaccatgaagagagaggagtggccacctaactaaccttcccagtttttgggagccaaacctagaccagaatgtaggtctaagtgactcccaatccagagctgtctccattaggccaggctctcaccccagctccaaaccaacttctaaaaacttgtccaagagtcctcctcttctttagaattggtaatcttggcaattaaattcagcgtagaaacactctcctgaacataatcagcatgctggttcttccttttctgttgccttgctcttcctaacagctcctcctttcgtctttgcaggctgcttctctgtcacaggaactcagggctcagtgctgtacttcatctccaaagtgtccctaaagcgcccatctgatcccatggctaactactccccaaattttctcctggactgaccttactgaatttagatttgtacatccaatacctgcttaacatatccactttgatgctcagtgggcacctcacacttgatctgtcaaacactgaatttctgtctctgttatgcacatacccaaactttccccaccatgtatttccccatctcaataaactgcaatagctcaagccaaaagcctaagattcagacctgaattctttcctttcctctctctcaaatgcaattcaacaattttcttaccttttattttttgttttggaatgaaggcacatataactgagctagtaataatgcttgattcataatacaccaccgatgttccatgcataactctcttattcatttgtccatgcatttattttgtttttgaatttttttaaaggggggcaaggtctacgttgcccaggttggaatatagtagctattcacaggtgaaatcatagcacactatagccttgaactggcctcaaggatcttcctatctcagactcccaagtagctgggactataagcacgcaccactacacccagctcatgtacttacttttaatgacaaatgaaccaccccaaaacccaccacctaacccagggactaaaacattaccagtgacttactcatagatttgctcctcctctacctctccagaggtaaccactatcttgaactttattactttttaaaagttttgtcacatatgtcaatgcctaaacagctgttcagttttagttgttcttgacttttataagaaaagtatcatgtcacatatagttttctcagaattgctttttcattctgagttattgtgctgcaagtagctggtattcattcattttgctgccatgtaataatcacccattctgtgaacacattacaccttcctaaaaatagacattttaatttattccagaacattcttatatgtgtgatctgggggacctgtgcaagcatttctcaagtatatactgaaaagtgaaattgctgacccatgggtatactttttttttttttttaaggtatgatcttactctgtcacccaaggtaagagtgcagtggcacaatcatgattcactgcagcctcaacctcctgggcttaagcaatccttccacctcagcttcccaagtagctgggaccacaggcatgcaccaccatgcccagctaattcaaaaaaatctttttgtgcagatgtggtctccctatgttgctcaagctggtcttgaactcttgggctcaagtgatcctcctaccttggcctcccaaagccaagaggcatgagccactgggcctggcccaacttttctagtgaatggtttttcacagtggatataccaattgatacccccatcagcaatatgtgagtgatcctaatgactaaaaccctctccaaaacttgactttgtgtttcttcattttcaccaatcgaatgaatttgaacatgtcattgtcatcttgatttacgttttcctgattgagagatgaaaacctcttaatgtttattggcccacatgcacttctaattgtgtggaaggcctggttcagtcttttgcctgtttttctgtgacactgtccttttttgttggtttgtagaatttctgcatacattcttgatactaagctattactagttataaatgttgcagatattgcctcacagtttgtagtttagctttagttttttttttagagacaaggtctccctatgttgcccaagttggacttgaacccctgggctcaagcaatcctcccacctcatcctcccaagttcatggacacagtgtgtgtgtgtgtgtgtgtgtgtgtgtgtgtgtaaatggagtttccctatttttcccaggcccgtctcaaactcctgggctcaagcagctcaagtaatccttctgcctctgcctcccaaagtgctgggattacaggcatgagccacaatgcctaactactgatgcacgatttctaaattaagaatttataatataccataacttatattcttttatggttatcttttatggtttttttttttcctgcttccagtttaagaagttcttcctaaagggagtaggatcaggaagataatcacattttctaaatatgtttcaatcacattttaatctataattccacatatagtttctacatcaagtcgtcatcctgttgcattaattttaaagagcatgcttctagtgtataaggttgaaaagcattcttccccttatagattactaaagatttattattaatgggtatactgattttctttagtcttactttttatttatcctttttaagtcatcaacaaactttttctgagtatttgattacctttctttcaaaccgtacagtatctcctggatttgtttctctttttatttaggtactttctccaaaagtgattttagtttgtacggaaaatcttctgaagctttgatggtacatattcttattaatgccctcacattagaataactattttcagaacataaaattgtaggttcaaagtttttttcaggttcaatttcacattcttgagctaggcatggtactgatggttttcaccataacatacaccaatgtccttttgtctgtgggctcccatccagcctggtggctgaagtcatctacaggtaagattgaccaaacctctgaacaggactgaaaaaaatgttatcttcagaaaaccagccctcttgtacactgctgctgtgaatacaaattgattaacttttctggatggcaatctagcaatgcagatcaaacatttaaaaatacatatatatctcgacacaattttatctccaggcatccacatgaaagaactccacaatgttcagaagtgtacagataaggatactcgtcacagcattataatatgaaaaataaactgaaaaccacctcatctccaaacacaattaaattatgttaaaattctataaacagggattaggatgtgtaggtttacccaagggaaaatatatttaatgtttaggtttaaaaagcaaaaaaaaagcctactttttgtttcaaaaatatgcatatgtaagtagaaaatatctgaaagctgaaaggctactatccaaaaatattaacagcagctttctctaaacagaaactaaagcagtttctcttttctttttgcttttctatacttattacatgtctaccacaaacctctttgttataatttctccagttgagtcagttttacaatttggaatgcagagatcaagtggttctataatcagcatatacttcgcacgtaccattcattcaatccacacccctttaaacccctttgacacacgtcaaactcatttacatctatgtccctccaatgacaatatagtggtcaacacatataaaacatgaatacactatatcaagacactcaggaatacatctctgggataaaatctgactgccttctattatattttaatgaataaccaaaataaagggattctttcagttacagagagcagaataattaaaatagtaactttcaaactttgtagcagcagaagtatttcttcaaataaaatcttttttgaaacccaatatagaaaacagataaaaataaagccattctagaggtgggggccttggaaagtgagtactatccactcagacttctttcttgcctctcacaaggaaggaagctactgtgtagtttgaaaattactatttaatacattctgctaaccctaaatgccatgtcagagctagaagagaaaatgtacacacattcaatctaacatttatttatttcaggttttttttttttttggcaactataaattacattcactagtacacctggaattcttcatagtgtgttcaactaaagaataagcaaacacagcatagatcagtttaaaagaaatcatggtacttcttagagcaatttgcaaaaggggaaaaaagtcttaggctcactccttggaaataaatatcaagtaaccataaaaatattcagccatttttcagttattcggggagttcaggcatggtcccacgcagagcatcagagttcctctttgaaataacccagctttgccaatgacatctcttttctcaactgcataacctcccaaaacatctgatcaacatcctgctgtttcacgagtccctgctgaatgtatcgaatgtatgtaaaaaagttacatacagaagtgatcctgtatctgcaaaaaggagaaatataataatagttgcttgagtcccctaatttaattctgtgtttacaggacttactctggccagtgagagcacatttttttggtcctccgcattcaactgcagaagctttcacaaaccggataggttgtaatcccactggttcaatgcttagagtattgttttccacagcctccagaacagctgaagccaactcactttttgagaatgttaaacatggaaagatatcttcctggtagattttgtctaagaaaggacacgtcctgtccattgtgggctcatccttccacaatcggaattcattatacaaggataagtcagcctctttgcagtcttttacaattggctgtatcacactgaggtcctgatgactgccactcatagcactgcttgtgcttttatttcttgtatgcccctttttaaaaggtgtctttccacctggcaaaggctcctgcgtaggtgatgttggagaactggacaatacaagtgtcttcaatgcagctacttcagcttgaagtacatcaatttttccttgtgcttcttttagctgtttttctgctgttgcctgcttgatatttgcttctctcaccattttatgagcttcctcaaatagactagctgtgagttcttccaattcctgtccaagttgatctcgcacttttgaaagcctctcacattcttcatcttttaacttcagttcctggctcagagggtcctacgcccacggaatctcgctgattgctagcacagcagtctgagatcaaactgcaaggcggcaacgaggctgggggagggacgcccgccattgcccaggcttgcttaggtaaacaaagcagccgggaagc

SEQ ID NO: 15989 - RNA, 6740 nt, Homo sapiens
  source 1..6740: mol_type = other RNA
gctgggattacaggcatgagccatcgcacctggccagtttttttttttttttttttttctaagtgcaatgggaagccactcaaagggctttaagcagggaagtgacattatctgattttcgttttataaagatccctgcggctgccgtcagtgattgtaggagggcaggagtggatgcaaggacagcagacattagtgcaggagttcaggtgaaagatgataatagcttgggcagagtggtagcagtggacatggagggaggtagacagatttaagatgtctcggagacagctgatggaatttgctgataactggaatgggagtgacaatgacaaataaaggaacctagaataagccccagaattttgcttaagcaactgagagttcagccatggcagatctgttaagcacaaaagttaaacacaaatacaaattcatactgcattggactcttttaagcagtgtcttatagaaaaaacattttatctagggaaaaatgcaacaacaaaaaccactgaaaacaaaagcctatgaataaaagcagacccgttttagactggatgcacaaaacaaaaacacacaggattcttgtggtggcgatgggagtaagtgaagacgtaacaggttgcaagttattttaaggactaagacccaatgttcagaaaccaaatcttgttcttccagtgtggatgcttagtcaaagactgtaaattgtcttcaagctgagagagaccatgaagagagaggagtggccacctaactaaccttcccagtttttgggagccaaacctagaccagaatgtaggtctaagtgactcccaatccagagctgtctccattaggccaggctctcaccccagctccaaaccaacttctaaaaacttgtccaagagtcctcctcttctttagaattggtaatcttggcaattaaattcagcgtagaaacactctcctgaacataatcagcatgctggttcttccttttctgttgccttgctcttcctaacagctcctcctttcgtctttgcaggctgcttctctgtcacaggaactcagggctcagtgctgtacttcatctccaaagtgtccctaaagcgcccatctgatcccatggctaactactccccaaattttctcctggactgaccttactgaatttagatttgtacatccaatacctgcttaacatatccactttgatgctcagtgggcacctcacacttgatctgtcaaacactgaatttctgtctctgttatgcacatacccaaactttccccaccatgtatttccccatctcaataaactgcaatagctcaagccaaaagcctaagattcagacctgaattctttcctttcctctctctcaaatgcaattcaacaattttcttaccttttattttttgttttggaatgaaggcacatataactgagctagtaataatgcttgattcataatacaccaccgatgttccatgcataactctcttattcatttgtccatgcatttattttgtttttgaatttttttaaaggggggcaaggtctacgttgcccaggttggaatatagtagctattcacaggtgaaatcatagcacactatagccttgaactggcctcaaggatcttcctatctcagactcccaagtagctgggactataagcacgcaccactacacccagctcatgtacttacttttaatgacaaatgaaccaccccaaaacccaccacctaacccagggactaaaacattaccagtgacttactcatagatttgctcctcctctacctctccagaggtaaccactatcttgaactttattactttttaaaagttttgtcacatatgtcaatgcctaaacagctgttcagttttagttgttcttgacttttataagaaaagtatcatgtcacatatagttttctcagaattgctttttcattctgagttattgtgctgcaagtagctggtattcattcattttgctgccatgtaataatcacccattctgtgaacacattacaccttcctaaaaatagacattttaatttattccagaacattcttatatgtgtgatctgggggacctgtgcaagcatttctcaagtatatactgaaaagtgaaattgctgacccatgggtatactttttttttttttttaaggtatgatcttactctgtcacccaaggtaagagtgcagtggcacaatcatgattcactgcagcctcaacctcctgggcttaagcaatccttccacctcagcttcccaagtagctgggaccacaggcatgcaccaccatgcccagctaattcaaaaaaatctttttgtgcagatgtggtctccctatgttgctcaagctggtcttgaactcttgggctcaagtgatcctcctaccttggcctcccaaagccaagaggcatgagccactgggcctggcccaacttttctagtgaatggtttttcacagtggatataccaattgatacccccatcagcaatatgtgagtgatcctaatgactaaaaccctctccaaaacttgactttgtgtttcttcattttcaccaatcgaatgaatttgaacatgtcattgtcatcttgatttacgttttcctgattgagagatgaaaacctcttaatgtttattggcccacatgcacttctaattgtgtggaaggcctggttcagtcttttgcctgtttttctgtgacactgtccttttttgttggtttgtagaatttctgcatacattcttgatactaagctattactagttataaatgttgcagatattgcctcacagtttgtagtttagctttagttttttttttagagacaaggtctccctatgttgcccaagttggacttgaacccctgggctcaagcaatcctcccacctcatcctcccaagttcatggacacagtgtgtgtgtgtgtgtgtgtgtgtgtgtgtgtgtaaatggagtttccctatttttcccaggcccgtctcaaactcctgggctcaagcagctcaagtaatccttctgcctctgcctcccaaagtgctgggattacaggcatgagccacaatgcctaactactgatgcacgatttctaaattaagaatttataatataccataacttatattcttttatggttatcttttatggtttttttttttcctgcttccagtttaagaagttcttcctaaagggagtaggatcaggaagataatcacattttctaaatatgtttcaatcacattttaatctataattccacatatagtttctacatcaagtcgtcatcctgttgcattaattttaaagagcatgcttctagtgtataaggttgaaaagcattcttccccttatagattactaaagatttattattaatgggtatactgattttctttagtcttactttttatttatcctttttaagtcatcaacaaactttttctgagtatttgattacctttctttcaaaccgtacagtatctcctggatttgtttctctttttatttaggtactttctccaaaagtgattttagtttgtacggaaaatcttctgaagctttgatggtacatattcttattaatgccctcacattagaataactattttcagaacataaaattgtaggttcaaagtttttttcaggttcaatttcacattcttgagctaggcatggtactgatggttttcaccataacatacaccaatgtccttttgtctgtgggctcccatccagcctggtggctgaagtcatctacaggtaagattgaccaaacctctgaacaggactgaaaaaaatgttatcttcagaaaaccagccctcttgtacactgctgctgtgaatacaaattgattaacttttctggatggcaatctagcaatgcagatcaaacatttaaaaatacatatatatctcgacacaattttatctccaggcatccacatgaaagaactccacaatgttcagaagtgtacagataaggatactcgtcacagcattataatatgaaaaataaactgaaaaccacctcatctccaaacacaattaaattatgttaaaattctataaacagggattaggatgtgtaggtttacccaagggaaaatatatttaatgtttaggtttaaaaagcaaaaaaaaagcctactttttgtttcaaaaatatgcatatgtaagtagaaaatatctgaaagctgaaaggctactatccaaaaatattaacagcagctttctctaaacagaaactaaagcagtttctcttttctttttgcttttctatacttattacatgtctaccacaaacctctttgttataatttctccagttgagtcagttttacaatttggaatgcagagatcaagtggttctataatcagcatatacttcgcacgtaccattcattcaatccacacccctttaaacccctttgacacacgtcaaactcatttacatctatgtccctccaatgacaatatagtggtcaacacatataaaacatgaatacactatatcaagacactcaggaatacatctctgggataaaatctgactgccttctattatattttaatgaataaccaaaataaagggattctttcagttacagagagcagaataattaaaatagtaactttcaaactttgtagcagcagaagtatttcttcaaataaaatcttttttgaaacccaatatagaaaacagataaaaataaagccattctagaggtgggggccttggaaagtgagtactatccactcagacttctttcttgcctctcacaaggaaggaagctactgtgtagtttgaaaattactatttaatacattctgctaaccctaaatgccatgtcagagctagaagagaaaatgtacacacattcaatctaacatttatttatttcaggttttttttttttttggcaactataaattacattcactagtacacctggaattcttcatagtgtgttcaactaaagaataagcaaacacagcatagatcagtttaaaagaaatcatggtacttcttagagcaatttgcaaaaggggaaaaaagtcttaggctcactccttggaaataaatatcaagtaaccataaaaatattcagccatttttcagttattcggggagttcaggcatggtcccacgcagagcatcagagttcctctttgaaataacccagctttgccaatgacatctcttttctcaactgcataacctcccaaaacatctgatcaacatcctgctgtttcacgagtccctgctgaatgtatcgaatgtatgtaaaaaagttacatacagaagtgatcctgtatctgcaaaaaggagaaatataataatagttgcttgagtcccctaatttaattctgtgtttacaggacttactctggccagtgagagcacatttttttggtcctccgcattcaactgcagaagctttcacaaaccggataggttgtaatcccactggttcaatgcttagagtattgttttccacagcctccagaacagctgaagccaatttttgagaatgttaaacatggaaagatatcttcctggtagattttgtctaagaaaggacacgtcctgtccattgtgggctcatccttccacaatcggaattcattatacaaggataagtcagcctctttgcagtcttttacaattggctgtatcacactgaggtcctgatgactgccactcatagcactgcttgtgcttttatttcttgtatgcccctttttaaaaggtgtctttccacctggcaaaggctcctgcgtaggtgatgttggagaactggacaatacaagtgtcttcaatgcagctacttcagcttgaagtacatcaatttttccttgtgcttcttttagctgtttttctgctgttgcctgcttgatatttgcttctctcaccattttatgagcttcctcaaatagactagctgtgagttcttccaattcctgtccaagttgatctcgcacttttgaaagcctctcacattcttcatcttttaacttcagttccctctgagcttttgcgagttcttcttttaatcgttcatagcccttttctctaacttccaaaacagatgggcttcgtaaacgagacagactatcagtactcaacccaaaaatatcatcactgccatcgcaagcctctgttatagtagcaccctgtaaaaactctctctctgcattatagttgtcctttcttgtagttaatttagttaatccagctgtgactccagaggtagagcaaggggctgggtctgtaacatgaaagctgatactagatatttccgcacaatttaaacgtctgggggatgaatacacgggttgtgtaggaagttcagaaacatctaatgcatttgcctggataggtacagaggataaagctgaagggtgtggccggtagatgacacttggtgaggtagtctgctcttgagttcctgattcatacacaccaagaaggtccggagaagtaggtgaagcaaggtttacttcatggaagccttccaagggatcattagccatagcaaaagcctcatcataagataacctgaagaacccaccgcggccgctgccggcgctcaggggcgctcacagagccgcagagagcgcgtcccgaagcagcgagaaacggaggaggacggcgagccctttccgctacactccacggcggcgggctcactacgccggcagccgccgagggaacgcgggactgcgcctgc

SEQ ID NO: 15990 - RNA, 6710 nt, Homo sapiens
  source 1..6710: mol_type = other RNA
gctgggattacaggcatgagccatcgcacctggccagtttttttttttttttttttttctaagtgcaatgggaagccactcaaagggctttaagcagggaagtgacattatctgattttcgttttataaagatccctgcggctgccgtcagtgattgtaggagggcaggagtggatgcaaggacagcagacattagtgcaggagttcaggtgaaagatgataatagcttgggcagagtggtagcagtggacatggagggaggtagacagatttaagatgtctcggagacagctgatggaatttgctgataactggaatgggagtgacaatgacaaataaaggaacctagaataagccccagaattttgcttaagcaactgagagttcagccatggcagatctgttaagcacaaaagttaaacacaaatacaaattcatactgcattggactcttttaagcagtgtcttatagaaaaaacattttatctagggaaaaatgcaacaacaaaaaccactgaaaacaaaagcctatgaataaaagcagacccgttttagactggatgcacaaaacaaaaacacacaggattcttgtggtggcgatgggagtaagtgaagacgtaacaggttgcaagttattttaaggactaagacccaatgttcagaaaccaaatcttgttcttccagtgtggatgcttagtcaaagactgtaaattgtcttcaagctgagagagaccatgaagagagaggagtggccacctaactaaccttcccagtttttgggagccaaacctagaccagaatgtaggtctaagtgactcccaatccagagctgtctccattaggccaggctctcaccccagctccaaaccaacttctaaaaacttgtccaagagtcctcctcttctttagaattggtaatcttggcaattaaattcagcgtagaaacactctcctgaacataatcagcatgctggttcttccttttctgttgccttgctcttcctaacagctcctcctttcgtctttgcaggctgcttctctgtcacaggaactcagggctcagtgctgtacttcatctccaaagtgtccctaaagcgcccatctgatcccatggctaactactccccaaattttctcctggactgaccttactgaatttagatttgtacatccaatacctgcttaacatatccactttgatgctcagtgggcacctcacacttgatctgtcaaacactgaatttctgtctctgttatgcacatacccaaactttccccaccatgtatttccccatctcaataaactgcaatagctcaagccaaaagcctaagattcagacctgaattctttcctttcctctctctcaaatgcaattcaacaattttcttaccttttattttttgttttggaatgaaggcacatataactgagctagtaataatgcttgattcataatacaccaccgatgttccatgcataactctcttattcatttgtccatgcatttattttgtttttgaatttttttaaaggggggcaaggtctacgttgcccaggttggaatatagtagctattcacaggtgaaatcatagcacactatagccttgaactggcctcaaggatcttcctatctcagactcccaagtagctgggactataagcacgcaccactacacccagctcatgtacttacttttaatgacaaatgaaccaccccaaaacccaccacctaacccagggactaaaacattaccagtgacttactcatagatttgctcctcctctacctctccagaggtaaccactatcttgaactttattactttttaaaagttttgtcacatatgtcaatgcctaaacagctgttcagttttagttgttcttgacttttataagaaaagtatcatgtcacatatagttttctcagaattgctttttcattctgagttattgtgctgcaagtagctggtattcattcattttgctgccatgtaataatcacccattctgtgaacacattacaccttcctaaaaatagacattttaatttattccagaacattcttatatgtgtgatctgggggacctgtgcaagcatttctcaagtatatactgaaaagtgaaattgctgacccatgggtatactttttttttttttttaaggtatgatcttactctgtcacccaaggtaagagtgcagtggcacaatcatgattcactgcagcctcaacctcctgggcttaagcaatccttccacctcagcttcccaagtagctgggaccacaggcatgcaccaccatgcccagctaattcaaaaaaatctttttgtgcagatgtggtctccctatgttgctcaagctggtcttgaactcttgggctcaagtgatcctcctaccttggcctcccaaagccaagaggcatgagccactgggcctggcccaacttttctagtgaatggtttttcacagtggatataccaattgatacccccatcagcaatatgtgagtgatcctaatgactaaaaccctctccaaaacttgactttgtgtttcttcattttcaccaatcgaatgaatttgaacatgtcattgtcatcttgatttacgttttcctgattgagagatgaaaacctcttaatgtttattggcccacatgcacttctaattgtgtggaaggcctggttcagtcttttgcctgtttttctgtgacactgtccttttttgttggtttgtagaatttctgcatacattcttgatactaagctattactagttataaatgttgcagatattgcctcacagtttgtagtttagctttagttttttttttagagacaaggtctccctatgttgcccaagttggacttgaacccctgggctcaagcaatcctcccacctcatcctcccaagttcatggacacagtgtgtgtgtgtgtgtgtgtgtgtgtgtgtgtgtaaatggagtttccctatttttcccaggcccgtctcaaactcctgggctcaagcagctcaagtaatccttctgcctctgcctcccaaagtgctgggattacaggcatgagccacaatgcctaactactgatgcacgatttctaaattaagaatttataatataccataacttatattcttttatggttatcttttatggtttttttttttcctgcttccagtttaagaagttcttcctaaagggagtaggatcaggaagataatcacattttctaaatatgtttcaatcacattttaatctataattccacatatagtttctacatcaagtcgtcatcctgttgcattaattttaaagagcatgcttctagtgtataaggttgaaaagcattcttccccttatagattactaaagatttattattaatgggtatactgattttctttagtcttactttttatttatcctttttaagtcatcaacaaactttttctgagtatttgattacctttctttcaaaccgtacagtatctcctggatttgtttctctttttatttaggtactttctccaaaagtgattttagtttgtacggaaaatcttctgaagctttgatggtacatattcttattaatgccctcacattagaataactattttcagaacataaaattgtaggttcaaagtttttttcaggttcaatttcacattcttgagctaggcatggtactgatggttttcaccataacatacaccaatgtccttttgtctgtgggctcccatccagcctggtggctgaagtcatctacaggtaagattgaccaaacctctgaacaggactgaaaaaaatgttatcttcagaaaaccagccctcttgtacactgctgctgtgaatacaaattgattaacttttctggatggcaatctagcaatgcagatcaaacatttaaaaatacatatatatctcgacacaattttatctccaggcatccacatgaaagaactccacaatgttcagaagtgtacagataaggatactcgtcacagcattataatatgaaaaataaactgaaaaccacctcatctccaaacacaattaaattatgttaaaattctataaacagggattaggatgtgtaggtttacccaagggaaaatatatttaatgtttaggtttaaaaagcaaaaaaaaagcctactttttgtttcaaaaatatgcatatgtaagtagaaaatatctgaaagctgaaaggctactatccaaaaatattaacagcagctttctctaaacagaaactaaagcagtttctcttttctttttgcttttctatacttattacatgtctaccacaaacctctttgttataatttctccagttgagtcagttttacaatttggaatgcagagatcaagtggttctataatcagcatatacttcgcacgtaccattcattcaatccacacccctttaaacccctttgacacacgtcaaactcatttacatctatgtccctccaatgacaatatagtggtcaacacatataaaacatgaatacactatatcaagacactcaggaatacatctctgggataaaatctgactgccttctattatattttaatgaataaccaaaataaagggattctttcagttacagagagcagaataattaaaatagtaactttcaaactttgtagcagcagaagtatttcttcaaataaaatcttttttgaaacccaatatagaaaacagataaaaataaagccattctagaggtgggggccttggaaagtgagtactatccactcagacttctttcttgcctctcacaaggaaggaagctactgtgtagtttgaaaattactatttaatacattctgctaaccctaaatgccatgtcagagctagaagagaaaatgtacacacattcaatctaacatttatttatttcaggttttttttttttttggcaactataaattacattcactagtacacctggaattcttcatagtgtgttcaactaaagaataagcaaacacagcatagatcagtttaaaagaaatcatggtacttcttagagcaatttgcaaaaggggaaaaaagtcttaggctcactccttggaaataaatatcaagtaaccataaaaatattcagccatttttcagttattcggggagttcaggcatggtcccacgcagagcatcagagttcctctttgaaataacccagctttgccaatgacatctcttttctcaactgcataacctcccaaaacatctgatcaacatcctgctgtttcacgagtccctgctgaatgtatcgaatgtatgtaaaaaagttacatacagaagtgatcctgtatctgcaaaaaggagaaatataataatagttgcttgagtcccctaatttaattctgtgtttacaggacttactctggccagtgagagcacatttttttggtcctccgcattcaactgcagaagctttcacaaaccggataggttgtaatcccactggttcaatgcttagagtattgttttccacagcctccagaacagctgaagccaatttttgagaatgttaaacatggaaagatatcttcctggtagattttgtctaagaaaggacacgtcctgtccattgtgggctcatccttccacaatcggaattcattatacaaggataagtcagcctctttgcagtcttttacaattggctgtatcacactgaggtcctgatgactgccactcatagcactgcttgtgcttttatttcttgtatgcccctttttaaaaggtgtctttccacctggcaaaggctcctgcgtaggtgatgttggagaactggacaatacaagtgtcttcaatgcagctacttcagcttgaagtacatcaatttttccttgtgcttcttttagctgtttttctgctgttgcctgcttgatatttgcttctctcaccattttatgagcttcctcaaatagactagctgtgagttcttccaattcctgtccaagttgatctcgcacttttgaaagcctctcacattcttcatcttttaacttcagttccctctgagcttttgcgagttcttcttttaatcgttcatagcccttttctctaacttccaaaacagatgggcttcgtaaacgagacagactatcagtactcaacccaaaaatatcatcactgccatcgcaagcctctgttatagtagcaccctgtaaaaactctctctctgcattatagttgtcctttcttgtagttaatttagttaatccagctgtgactccagaggtagagcaaggggctgggtctgtaacatgaaagctgatactagatatttccgcacaatttaaacgtctgggggatgaatacacgggttgtgtaggaagttcagaaacatctaatgcatttgcctggataggtacagaggataaagctgaagggtgtggccggtagatgacacttggtgaggtagtctgctcttgagttcctgattcatacacaccaagaaggtccggagaagtaggtgaagcaaggtttacttcatggaagccttccaagggatcattagccatagcaaaagcctcatcataagataacctgagactccgcggccatatacaccttacgacgtgtgtgtgtgtggcgggagatgggaggggaggaatcctgtagaacccagatcccatcattccagcaactgccagagcgttcgagaatgtcatgtctgtacctgtcttct

SEQ ID NO: 15991 - RNA, 6597 nt, Homo sapiens
  source 1..6597: mol_type = other RNA
gctgggattacaggcatgagccatcgcacctggccagtttttttttttttttttttttctaagtgcaatgggaagccactcaaagggctttaagcagggaagtgacattatctgattttcgttttataaagatccctgcggctgccgtcagtgattgtaggagggcaggagtggatgcaaggacagcagacattagtgcaggagttcaggtgaaagatgataatagcttgggcagagtggtagcagtggacatggagggaggtagacagatttaagatgtctcggagacagctgatggaatttgctgataactggaatgggagtgacaatgacaaataaaggaacctagaataagccccagaattttgcttaagcaactgagagttcagccatggcagatctgttaagcacaaaagttaaacacaaatacaaattcatactgcattggactcttttaagcagtgtcttatagaaaaaacattttatctagggaaaaatgcaacaacaaaaaccactgaaaacaaaagcctatgaataaaagcagacccgttttagactggatgcacaaaacaaaaacacacaggattcttgtggtggcgatgggagtaagtgaagacgtaacaggttgcaagttattttaaggactaagacccaatgttcagaaaccaaatcttgttcttccagtgtggatgcttagtcaaagactgtaaattgtcttcaagctgagagagaccatgaagagagaggagtggccacctaactaaccttcccagtttttgggagccaaacctagaccagaatgtaggtctaagtgactcccaatccagagctgtctccattaggccaggctctcaccccagctccaaaccaacttctaaaaacttgtccaagagtcctcctcttctttagaattggtaatcttggcaattaaattcagcgtagaaacactctcctgaacataatcagcatgctggttcttccttttctgttgccttgctcttcctaacagctcctcctttcgtctttgcaggctgcttctctgtcacaggaactcagggctcagtgctgtacttcatctccaaagtgtccctaaagcgcccatctgatcccatggctaactactccccaaattttctcctggactgaccttactgaatttagatttgtacatccaatacctgcttaacatatccactttgatgctcagtgggcacctcacacttgatctgtcaaacactgaatttctgtctctgttatgcacatacccaaactttccccaccatgtatttccccatctcaataaactgcaatagctcaagccaaaagcctaagattcagacctgaattctttcctttcctctctctcaaatgcaattcaacaattttcttaccttttattttttgttttggaatgaaggcacatataactgagctagtaataatgcttgattcataatacaccaccgatgttccatgcataactctcttattcatttgtccatgcatttattttgtttttgaatttttttaaaggggggcaaggtctacgttgcccaggttggaatatagtagctattcacaggtgaaatcatagcacactatagccttgaactggcctcaaggatcttcctatctcagactcccaagtagctgggactataagcacgcaccactacacccagctcatgtacttacttttaatgacaaatgaaccaccccaaaacccaccacctaacccagggactaaaacattaccagtgacttactcatagatttgctcctcctctacctctccagaggtaaccactatcttgaactttattactttttaaaagttttgtcacatatgtcaatgcctaaacagctgttcagttttagttgttcttgacttttataagaaaagtatcatgtcacatatagttttctcagaattgctttttcattctgagttattgtgctgcaagtagctggtattcattcattttgctgccatgtaataatcacccattctgtgaacacattacaccttcctaaaaatagacattttaatttattccagaacattcttatatgtgtgatctgggggacctgtgcaagcatttctcaagtatatactgaaaagtgaaattgctgacccatgggtatactttttttttttttttaaggtatgatcttactctgtcacccaaggtaagagtgcagtggcacaatcatgattcactgcagcctcaacctcctgggcttaagcaatccttccacctcagcttcccaagtagctgggaccacaggcatgcaccaccatgcccagctaattcaaaaaaatctttttgtgcagatgtggtctccctatgttgctcaagctggtcttgaactcttgggctcaagtgatcctcctaccttggcctcccaaagccaagaggcatgagccactgggcctggcccaacttttctagtgaatggtttttcacagtggatataccaattgatacccccatcagcaatatgtgagtgatcctaatgactaaaaccctctccaaaacttgactttgtgtttcttcattttcaccaatcgaatgaatttgaacatgtcattgtcatcttgatttacgttttcctgattgagagatgaaaacctcttaatgtttattggcccacatgcacttctaattgtgtggaaggcctggttcagtcttttgcctgtttttctgtgacactgtccttttttgttggtttgtagaatttctgcatacattcttgatactaagctattactagttataaatgttgcagatattgcctcacagtttgtagtttagctttagttttttttttagagacaaggtctccctatgttgcccaagttggacttgaacccctgggctcaagcaatcctcccacctcatcctcccaagttcatggacacagtgtgtgtgtgtgtgtgtgtgtgtgtgtgtgtgtaaatggagtttccctatttttcccaggcccgtctcaaactcctgggctcaagcagctcaagtaatccttctgcctctgcctcccaaagtgctgggattacaggcatgagccacaatgcctaactactgatgcacgatttctaaattaagaatttataatataccataacttatattcttttatggttatcttttatggtttttttttttcctgcttccagtttaagaagttcttcctaaagggagtaggatcaggaagataatcacattttctaaatatgtttcaatcacattttaatctataattccacatatagtttctacatcaagtcgtcatcctgttgcattaattttaaagagcatgcttctagtgtataaggttgaaaagcattcttccccttatagattactaaagatttattattaatgggtatactgattttctttagtcttactttttatttatcctttttaagtcatcaacaaactttttctgagtatttgattacctttctttcaaaccgtacagtatctcctggatttgtttctctttttatttaggtactttctccaaaagtgattttagtttgtacggaaaatcttctgaagctttgatggtacatattcttattaatgccctcacattagaataactattttcagaacataaaattgtaggttcaaagtttttttcaggttcaatttcacattcttgagctaggcatggtactgatggttttcaccataacatacaccaatgtccttttgtctgtgggctcccatccagcctggtggctgaagtcatctacaggtaagattgaccaaacctctgaacaggactgaaaaaaatgttatcttcagaaaaccagccctcttgtacactgctgctgtgaatacaaattgattaacttttctggatggcaatctagcaatgcagatcaaacatttaaaaatacatatatatctcgacacaattttatctccaggcatccacatgaaagaactccacaatgttcagaagtgtacagataaggatactcgtcacagcattataatatgaaaaataaactgaaaaccacctcatctccaaacacaattaaattatgttaaaattctataaacagggattaggatgtgtaggtttacccaagggaaaatatatttaatgtttaggtttaaaaagcaaaaaaaaagcctactttttgtttcaaaaatatgcatatgtaagtagaaaatatctgaaagctgaaaggctactatccaaaaatattaacagcagctttctctaaacagaaactaaagcagtttctcttttctttttgcttttctatacttattacatgtctaccacaaacctctttgttataatttctccagttgagtcagttttacaatttggaatgcagagatcaagtggttctataatcagcatatacttcgcacgtaccattcattcaatccacacccctttaaacccctttgacacacgtcaaactcatttacatctatgtccctccaatgacaatatagtggtcaacacatataaaacatgaatacactatatcaagacactcaggaatacatctctgggataaaatctgactgccttctattatattttaatgaataaccaaaataaagggattctttcagttacagagagcagaataattaaaatagtaactttcaaactttgtagcagcagaagtatttcttcaaataaaatcttttttgaaacccaatatagaaaacagataaaaataaagccattctagaggtgggggccttggaaagtgagtactatccactcagacttctttcttgcctctcacaaggaaggaagctactgtgtagtttgaaaattactatttaatacattctgctaaccctaaatgccatgtcagagctagaagagaaaatgtacacacattcaatctaacatttatttatttcaggttttttttttttttggcaactataaattacattcactagtacacctggaattcttcatagtgtgttcaactaaagaataagcaaacacagcatagatcagtttaaaagaaatcatggtacttcttagagcaatttgcaaaaggggaaaaaagtcttaggctcactccttggaaataaatatcaagtaaccataaaaatattcagccatttttcagttattcggggagttcaggcatggtcccacgcagagcatcagagttcctctttgaaataacccagctttgccaatgacatctcttttctcaactgcataacctcccaaaacatctgatcaacatcctgctgtttcacgagtccctgctgaatgtatcgaatgtatgtaaaaaagttacatacagaagtgatcctgtatctgcaaaaaggagaaatataataatagttgcttgagtcccctaatttaattctgtgtttacaggacttactctggccagtgagagcacatttttttttgagaatgttaaacatggaaagatatcttcctggtagattttgtctaagaaaggacacgtcctgtccattgtgggctcatccttccacaatcggaattcattatacaaggataagtcagcctctttgcagtcttttacaattggctgtatcacactgaggtcctgatgactgccactcatagcactgcttgtgcttttatttcttgtatgcccctttttaaaaggtgtctttccacctggcaaaggctcctgcgtaggtgatgttggagaactggacaatacaagtgtcttcaatgcagctacttcagcttgaagtacatcaatttttccttgtgcttcttttagctgtttttctgctgttgcctgcttgatatttgcttctctcaccattttatgagcttcctcaaatagactagctgtgagttcttccaattcctgtccaagttgatctcgcacttttgaaagcctctcacattcttcatcttttaacttcagttccctctgagcttttgcgagttcttcttttaatcgttcatagcccttttctctaacttccaaaacagatgggcttcgtaaacgagacagactatcagtactcaacccaaaaatatcatcactgccatcgcaagcctctgttatagtagcaccctgtaaaaactctctctctgcattatagttgtcctttcttgtagttaatttagttaatccagctgtgactccagaggtagagcaaggggctgggtctgtaacatgaaagctgatactagatatttccgcacaatttaaacgtctgggggatgaatacacgggttgtgtaggaagttcagaaacatctaatgcatttgcctggataggtacagaggataaagctgaagggtgtggccggtagatgacacttggtgaggtagtctgctcttgagttcctgattcatacacaccaagaaggtccggagaagtaggtgaagcaaggtttacttcatggaagccttccaagggatcattagccatagcaaaagcctcatcataagataacctgagactccgcggccatatacaccttacgacgtgtgtgtgtgtggcgggagatgggaggggaggaatcctgtagaacccagatcccatcattccagcaactgccagagcgttcgagaatgtcatgtctgtacctgtcttct

SEQ ID NO: 15992 - RNA, 6962 nt, Homo sapiens
  source 1..6962: mol_type = other RNA
gctgggattacaggcatgagccatcgcacctggccagtttttttttttttttttttttctaagtgcaatgggaagccactcaaagggctttaagcagggaagtgacattatctgattttcgttttataaagatccctgcggctgccgtcagtgattgtaggagggcaggagtggatgcaaggacagcagacattagtgcaggagttcaggtgaaagatgataatagcttgggcagagtggtagcagtggacatggagggaggtagacagatttaagatgtctcggagacagctgatggaatttgctgataactggaatgggagtgacaatgacaaataaaggaacctagaataagccccagaattttgcttaagcaactgagagttcagccatggcagatctgttaagcacaaaagttaaacacaaatacaaattcatactgcattggactcttttaagcagtgtcttatagaaaaaacattttatctagggaaaaatgcaacaacaaaaaccactgaaaacaaaagcctatgaataaaagcagacccgttttagactggatgcacaaaacaaaaacacacaggattcttgtggtggcgatgggagtaagtgaagacgtaacaggttgcaagttattttaaggactaagacccaatgttcagaaaccaaatcttgttcttccagtgtggatgcttagtcaaagactgtaaattgtcttcaagctgagagagaccatgaagagagaggagtggccacctaactaaccttcccagtttttgggagccaaacctagaccagaatgtaggtctaagtgactcccaatccagagctgtctccattaggccaggctctcaccccagctccaaaccaacttctaaaaacttgtccaagagtcctcctcttctttagaattggtaatcttggcaattaaattcagcgtagaaacactctcctgaacataatcagcatgctggttcttccttttctgttgccttgctcttcctaacagctcctcctttcgtctttgcaggctgcttctctgtcacaggaactcagggctcagtgctgtacttcatctccaaagtgtccctaaagcgcccatctgatcccatggctaactactccccaaattttctcctggactgaccttactgaatttagatttgtacatccaatacctgcttaacatatccactttgatgctcagtgggcacctcacacttgatctgtcaaacactgaatttctgtctctgttatgcacatacccaaactttccccaccatgtatttccccatctcaataaactgcaatagctcaagccaaaagcctaagattcagacctgaattctttcctttcctctctctcaaatgcaattcaacaattttcttaccttttattttttgttttggaatgaaggcacatataactgagctagtaataatgcttgattcataatacaccaccgatgttccatgcataactctcttattcatttgtccatgcatttattttgtttttgaatttttttaaaggggggcaaggtctacgttgcccaggttggaatatagtagctattcacaggtgaaatcatagcacactatagccttgaactggcctcaaggatcttcctatctcagactcccaagtagctgggactataagcacgcaccactacacccagctcatgtacttacttttaatgacaaatgaaccaccccaaaacccaccacctaacccagggactaaaacattaccagtgacttactcatagatttgctcctcctctacctctccagaggtaaccactatcttgaactttattactttttaaaagttttgtcacatatgtcaatgcctaaacagctgttcagttttagttgttcttgacttttataagaaaagtatcatgtcacatatagttttctcagaattgctttttcattctgagttattgtgctgcaagtagctggtattcattcattttgctgccatgtaataatcacccattctgtgaacacattacaccttcctaaaaatagacattttaatttattccagaacattcttatatgtgtgatctgggggacctgtgcaagcatttctcaagtatatactgaaaagtgaaattgctgacccatgggtatactttttttttttttttaaggtatgatcttactctgtcacccaaggtaagagtgcagtggcacaatcatgattcactgcagcctcaacctcctgggcttaagcaatccttccacctcagcttcccaagtagctgggaccacaggcatgcaccaccatgcccagctaattcaaaaaaatctttttgtgcagatgtggtctccctatgttgctcaagctggtcttgaactcttgggctcaagtgatcctcctaccttggcctcccaaagccaagaggcatgagccactgggcctggcccaacttttctagtgaatggtttttcacagtggatataccaattgatacccccatcagcaatatgtgagtgatcctaatgactaaaaccctctccaaaacttgactttgtgtttcttcattttcaccaatcgaatgaatttgaacatgtcattgtcatcttgatttacgttttcctgattgagagatgaaaacctcttaatgtttattggcccacatgcacttctaattgtgtggaaggcctggttcagtcttttgcctgtttttctgtgacactgtccttttttgttggtttgtagaatttctgcatacattcttgatactaagctattactagttataaatgttgcagatattgcctcacagtttgtagtttagctttagttttttttttagagacaaggtctccctatgttgcccaagttggacttgaacccctgggctcaagcaatcctcccacctcatcctcccaagttcatggacacagtgtgtgtgtgtgtgtgtgtgtgtgtgtgtgtgtaaatggagtttccctatttttcccaggcccgtctcaaactcctgggctcaagcagctcaagtaatccttctgcctctgcctcccaaagtgctgggattacaggcatgagccacaatgcctaactactgatgcacgatttctaaattaagaatttataatataccataacttatattcttttatggttatcttttatggtttttttttttcctgcttccagtttaagaagttcttcctaaagggagtaggatcaggaagataatcacattttctaaatatgtttcaatcacattttaatctataattccacatatagtttctacatcaagtcgtcatcctgttgcattaattttaaagagcatgcttctagtgtataaggttgaaaagcattcttccccttatagattactaaagatttattattaatgggtatactgattttctttagtcttactttttatttatcctttttaagtcatcaacaaactttttctgagtatttgattacctttctttcaaaccgtacagtatctcctggatttgtttctctttttatttaggtactttctccaaaagtgattttagtttgtacggaaaatcttctgaagctttgatggtacatattcttattaatgccctcacattagaataactattttcagaacataaaattgtaggttcaaagtttttttcaggttcaatttcacattcttgagctaggcatggtactgatggttttcaccataacatacaccaatgtccttttgtctgtgggctcccatccagcctggtggctgaagtcatctacaggtaagattgaccaaacctctgaacaggactgaaaaaaatgttatcttcagaaaaccagccctcttgtacactgctgctgtgaatacaaattgattaacttttctggatggcaatctagcaatgcagatcaaacatttaaaaatacatatatatctcgacacaattttatctccaggcatccacatgaaagaactccacaatgttcagaagtgtacagataaggatactcgtcacagcattataatatgaaaaataaactgaaaaccacctcatctccaaacacaattaaattatgttaaaattctataaacagggattaggatgtgtaggtttacccaagggaaaatatatttaatgtttaggtttaaaaagcaaaaaaaaagcctactttttgtttcaaaaatatgcatatgtaagtagaaaatatctgaaagctgaaaggctactatccaaaaatattaacagcagctttctctaaacagaaactaaagcagtttctcttttctttttgcttttctatacttattacatgtctaccacaaacctctttgttataatttctccagttgagtcagttttacaatttggaatgcagagatcaagtggttctataatcagcatatacttcgcacgtaccattcattcaatccacacccctttaaacccctttgacacacgtcaaactcatttacatctatgtccctccaatgacaatatagtggtcaacacatataaaacatgaatacactatatcaagacactcaggaatacatctctgggataaaatctgactgccttctattatattttaatgaataaccaaaataaagggattctttcagttacagagagcagaataattaaaatagtaactttcaaactttgtagcagcagaagtatttcttcaaataaaatcttttttgaaacccaatatagaaaacagataaaaataaagccattctagaggtgggggccttggaaagtgagtactatccactcagacttctttcttgcctctcacaaggaaggaagctactgtgtagtttgaaaattactatttaatacattctgctaaccctaaatgccatgtcagagctagaagagaaaatgtacacacattcaatctaacatttatttatttcaggttttttttttttttggcaactataaattacattcactagtacacctggaattcttcatagtgtgttcaactaaagaataagcaaacacagcatagatcagtttaaaagaaatcatggtacttcttagagcaatttgcaaaaggggaaaaaagtcttaggctcactccttggaaataaatatcaagtaaccataaaaatattcagccatttttcagttattcggggagttcaggcatggtcccacgcagagcatcagagttcctctttgaaataacccagctttgccaatgacatctcttttctcaactgcataacctcccaaaacatctgatcaacatcctgctgtttcacgagtccctgctgaatgtatcgaatgtatgtaaaaaagttacatacagaagtgattttggtcctccgcattcaactgcagaagctttcacaaaccggataggttgtaatcccactggttcaatgcttagagtattgttttccacagcctccagaacagctgaagccaactcactttttgagaatgttaaacatggaaagatatcttcctggtagattttgtctaagaaaggacacgtcctgtccattgtgggctcatccttccacaatcggaattcattatacaaggataagtcagcctctttgcagtcttttacaattggctgtatcacactgaggtcctgatgactgccactcatagcactgcttgtgcttttatttcttgtatgcccctttttaaaaggtgtctttccacctggcaaaggctcctgcgtaggtgatgttggagaactggacaatacaagtgtcttcaatgcagctacttcagcttgaagtacatcaatttttccttgtgcttcttttagctgtttttctgctgttgcctgcttgatatttgcttctctcaccattttatgagcttcctcaaatagactagctgtgagttcttccaattcctgtccaagttgatctcgcacttttgaaagcctctcacattcttcatcttttaacttcagttccctctgagcttttgcgagttcttcttttaatcgttcatagcccttttctctaacttccaaaacagatgggcttcgtaaacgagacagactatcagtactcaacccaaaaatatcatcactgccatcgcaagcctctgttatagtagcaccctgtaaaaactctctctctgcattatagttgtcctttcttgtagttaatttagttaatccagctgtgactccagaggtagagcaaggggctgggtctgtaacatgaaagctgatactagatatttccgcacaatttaaacgtctgggggatgaatacacgggttgtgtaggaagttcagaaacatctaatgcatttgcctggataggtacagaggataaagctgaagggtgtggccggtagatgacacttggtgaggtagtctgctcttgagttcctgattcatacacaccaagaaggtccggagaagtaggtgaagcaaggtttacttcatggaagccttccaagggatcattagccatagcaaaagcctcatcataagataaccctttcatcttttttaatcccataacaaccggcaactcttcacatgctgcgacttccacccagcatcatcacttctggagccagtaagctcgcgcttcctgggcggtcggggcgagttgtcaacgctgggagggcagagccatgcaatcccacccgtgcagttcgtctcaactcccccgaacacaagtctggcggcacggagctgcctacttgggcgcgactccgggcgcctgcccggaatttcccaccaggtttcaccgaaacctcccgagggtgacctctacgcctcagcacggtgcctcgcgcgtagtttcctaagactgggacacgaaaccaccccaggtccacagccctgccgcgcggcgtccggtgttgtgagctgcttccgacttgttcgggaactctctcttcatcctcttcgcgaccgcggccctccgctcccggccgcgcccgcccgccgccaggtaacccgctggactcgggctccct

SEQ ID NO: 15993 - RNA, 6645 nt, Homo sapiens
  source 1..6645: mol_type = other RNA
gctgggattacaggcatgagccatcgcacctggccagtttttttttttttttttttttctaagtgcaatgggaagccactcaaagggctttaagcagggaagtgacattatctgattttcgttttataaagatccctgcggctgccgtcagtgattgtaggagggcaggagtggatgcaaggacagcagacattagtgcaggagttcaggtgaaagatgataatagcttgggcagagtggtagcagtggacatggagggaggtagacagatttaagatgtctcggagacagctgatggaatttgctgataactggaatgggagtgacaatgacaaataaaggaacctagaataagccccagaattttgcttaagcaactgagagttcagccatggcagatctgttaagcacaaaagttaaacacaaatacaaattcatactgcattggactcttttaagcagtgtcttatagaaaaaacattttatctagggaaaaatgcaacaacaaaaaccactgaaaacaaaagcctatgaataaaagcagacccgttttagactggatgcacaaaacaaaaacacacaggattcttgtggtggcgatgggagtaagtgaagacgtaacaggttgcaagttattttaaggactaagacccaatgttcagaaaccaaatcttgttcttccagtgtggatgcttagtcaaagactgtaaattgtcttcaagctgagagagaccatgaagagagaggagtggccacctaactaaccttcccagtttttgggagccaaacctagaccagaatgtaggtctaagtgactcccaatccagagctgtctccattaggccaggctctcaccccagctccaaaccaacttctaaaaacttgtccaagagtcctcctcttctttagaattggtaatcttggcaattaaattcagcgtagaaacactctcctgaacataatcagcatgctggttcttccttttctgttgccttgctcttcctaacagctcctcctttcgtctttgcaggctgcttctctgtcacaggaactcagggctcagtgctgtacttcatctccaaagtgtccctaaagcgcccatctgatcccatggctaactactccccaaattttctcctggactgaccttactgaatttagatttgtacatccaatacctgcttaacatatccactttgatgctcagtgggcacctcacacttgatctgtcaaacactgaatttctgtctctgttatgcacatacccaaactttccccaccatgtatttccccatctcaataaactgcaatagctcaagccaaaagcctaagattcagacctgaattctttcctttcctctctctcaaatgcaattcaacaattttcttaccttttattttttgttttggaatgaaggcacatataactgagctagtaataatgcttgattcataatacaccaccgatgttccatgcataactctcttattcatttgtccatgcatttattttgtttttgaatttttttaaaggggggcaaggtctacgttgcccaggttggaatatagtagctattcacaggtgaaatcatagcacactatagccttgaactggcctcaaggatcttcctatctcagactcccaagtagctgggactataagcacgcaccactacacccagctcatgtacttacttttaatgacaaatgaaccaccccaaaacccaccacctaacccagggactaaaacattaccagtgacttactcatagatttgctcctcctctacctctccagaggtaaccactatcttgaactttattactttttaaaagttttgtcacatatgtcaatgcctaaacagctgttcagttttagttgttcttgacttttataagaaaagtatcatgtcacatatagttttctcagaattgctttttcattctgagttattgtgctgcaagtagctggtattcattcattttgctgccatgtaataatcacccattctgtgaacacattacaccttcctaaaaatagacattttaatttattccagaacattcttatatgtgtgatctgggggacctgtgcaagcatttctcaagtatatactgaaaagtgaaattgctgacccatgggtatactttttttttttttttaaggtatgatcttactctgtcacccaaggtaagagtgcagtggcacaatcatgattcactgcagcctcaacctcctgggcttaagcaatccttccacctcagcttcccaagtagctgggaccacaggcatgcaccaccatgcccagctaattcaaaaaaatctttttgtgcagatgtggtctccctatgttgctcaagctggtcttgaactcttgggctcaagtgatcctcctaccttggcctcccaaagccaagaggcatgagccactgggcctggcccaacttttctagtgaatggtttttcacagtggatataccaattgatacccccatcagcaatatgtgagtgatcctaatgactaaaaccctctccaaaacttgactttgtgtttcttcattttcaccaatcgaatgaatttgaacatgtcattgtcatcttgatttacgttttcctgattgagagatgaaaacctcttaatgtttattggcccacatgcacttctaattgtgtggaaggcctggttcagtcttttgcctgtttttctgtgacactgtccttttttgttggtttgtagaatttctgcatacattcttgatactaagctattactagttataaatgttgcagatattgcctcacagtttgtagtttagctttagttttttttttagagacaaggtctccctatgttgcccaagttggacttgaacccctgggctcaagcaatcctcccacctcatcctcccaagttcatggacacagtgtgtgtgtgtgtgtgtgtgtgtgtgtgtgtgtaaatggagtttccctatttttcccaggcccgtctcaaactcctgggctcaagcagctcaagtaatccttctgcctctgcctcccaaagtgctgggattacaggcatgagccacaatgcctaactactgatgcacgatttctaaattaagaatttataatataccataacttatattcttttatggttatcttttatggtttttttttttcctgcttccagtttaagaagttcttcctaaagggagtaggatcaggaagataatcacattttctaaatatgtttcaatcacattttaatctataattccacatatagtttctacatcaagtcgtcatcctgttgcattaattttaaagagcatgcttctagtgtataaggttgaaaagcattcttccccttatagattactaaagatttattattaatgggtatactgattttctttagtcttactttttatttatcctttttaagtcatcaacaaactttttctgagtatttgattacctttctttcaaaccgtacagtatctcctggatttgtttctctttttatttaggtactttctccaaaagtgattttagtttgtacggaaaatcttctgaagctttgatggtacatattcttattaatgccctcacattagaataactattttcagaacataaaattgtaggttcaaagtttttttcaggttcaatttcacattcttgagctaggcatggtactgatggttttcaccataacatacaccaatgtccttttgtctgtgggctcccatccagcctggtggctgaagtcatctacaggtaagattgaccaaacctctgaacaggactgaaaaaaatgttatcttcagaaaaccagccctcttgtacactgctgctgtgaatacaaattgattaacttttctggatggcaatctagcaatgcagatcaaacatttaaaaatacatatatatctcgacacaattttatctccaggcatccacatgaaagaactccacaatgttcagaagtgtacagataaggatactcgtcacagcattataatatgaaaaataaactgaaaaccacctcatctccaaacacaattaaattatgttaaaattctataaacagggattaggatgtgtaggtttacccaagggaaaatatatttaatgtttaggtttaaaaagcaaaaaaaaagcctactttttgtttcaaaaatatgcatatgtaagtagaaaatatctgaaagctgaaaggctactatccaaaaatattaacagcagctttctctaaacagaaactaaagcagtttctcttttctttttgcttttctatacttattacatgtctaccacaaacctctttgttataatttctccagttgagtcagttttacaatttggaatgcagagatcaagtggttctataatcagcatatacttcgcacgtaccattcattcaatccacacccctttaaacccctttgacacacgtcaaactcatttacatctatgtccctccaatgacaatatagtggtcaacacatataaaacatgaatacactatatcaagacactcaggaatacatctctgggataaaatctgactgccttctattatattttaatgaataaccaaaataaagggattctttcagttacagagagcagaataattaaaatagtaactttcaaactttgtagcagcagaagtatttcttcaaataaaatcttttttgaaacccaatatagaaaacagataaaaataaagccattctagaggtgggggccttggaaagtgagtactatccactcagacttctttcttgcctctcacaaggaaggaagctactgtgtagtttgaaaattactatttaatacattctgctaaccctaaatgccatgtcagagctagaagagaaaatgtacacacattcaatctaacatttatttatttcaggttttttttttttttggcaactataaattacattcactagtacacctggaattcttcatagtgtgttcaactaaagaataagcaaacacagcatagatcagtttaaaagaaatcatggtacttcttagagcaatttgcaaaaggggaaaaaagtcttaggctcactccttggaaataaatatcaagtaaccataaaaatattcagccatttttcagttattcggggagttcaggcatggtcccacgcagagcatcagagttcctctttgaaataacccagctttgccaatgacatctcttttctcaactgcataacctcccaaaacatctgatcaacatcctgctgtttcacgagtccctgctgaatgtatcgaatgtatgtaaaaaagttacatacagaagtgattttggtcctccgcattcaactgcagaagctttcacaaaccggataggttgtaatcccactggttcaatgcttagagtattgttttccacagcctccagaacagctgaagccaactcactttttgagaatgttaaacatggaaagatatcttcctggtagattttgtctaagaaaggacacgtcctgtccattgtgggctcatccttccacaatcggaattcattatacaaggataagtcagcctctttgcagtcttttacaattggctgtatcacactgaggtcctgatgactgccactcatagcactgcttgtgcttttatttcttgtatgcccctttttaaaaggtgtctttccacctggcaaaggctcctgcgtaggtgatgttggagaactggacaatacaagtgtcttcaatgcagctacttcagcttgaagtacatcaatttttccttgtgcttcttttagctgtttttctgctgttgcctgcttgatatttgcttctctcaccattttatgagcttcctcaaatagactagctgtgagttcttccaattcctgtccaagttgatctcgcacttttgaaagcctctcacattcttcatcttttaacttcagttccctctgagcttttgcgagttcttcttttaatcgttcatagcccttttctctaacttccaaaacagatgggcttcgtaaacgagacagactatcagtactcaacccaaaaatatcatcactgccatcgcaagcctctgttatagtagcaccctgtaaaaactctctctctgcattatagttgtcctttcttgtagttaatttagttaatccagctgtgactccagaggtagagcaaggggctgggtctgtaacatgaaagctgatactagatatttccgcacaatttaaacgtctgggggatgaatacacgggttgtgtaggaagttcagaaacatctaatgcatttgcctggataggtacagaggataaagctgaagggtgtggccggtagatgacacttggtgaggtagtctgctcttgagttcctgattcatacacaccaagaaggtccggagaagtaggtgaagcaaggtttacttcatggaagccttccaagggatcattagccatagcaaaagcctcatcataagataacctgaagaacccaccgcggccgctgccggcgctcaggggcgctcacagagccgcagagagcgcgtcccgaagcagcgagaaacggaggaggacggcgagccctttccgctacactccacggcggcgggctcactacgccggcagccgccgagggaacgcgggactgcgcctgc

SEQ ID NO: 15994 - RNA, 6615 nt, Homo sapiens
  source 1..6615: mol_type = other RNA
gctgggattacaggcatgagccatcgcacctggccagtttttttttttttttttttttctaagtgcaatgggaagccactcaaagggctttaagcagggaagtgacattatctgattttcgttttataaagatccctgcggctgccgtcagtgattgtaggagggcaggagtggatgcaaggacagcagacattagtgcaggagttcaggtgaaagatgataatagcttgggcagagtggtagcagtggacatggagggaggtagacagatttaagatgtctcggagacagctgatggaatttgctgataactggaatgggagtgacaatgacaaataaaggaacctagaataagccccagaattttgcttaagcaactgagagttcagccatggcagatctgttaagcacaaaagttaaacacaaatacaaattcatactgcattggactcttttaagcagtgtcttatagaaaaaacattttatctagggaaaaatgcaacaacaaaaaccactgaaaacaaaagcctatgaataaaagcagacccgttttagactggatgcacaaaacaaaaacacacaggattcttgtggtggcgatgggagtaagtgaagacgtaacaggttgcaagttattttaaggactaagacccaatgttcagaaaccaaatcttgttcttccagtgtggatgcttagtcaaagactgtaaattgtcttcaagctgagagagaccatgaagagagaggagtggccacctaactaaccttcccagtttttgggagccaaacctagaccagaatgtaggtctaagtgactcccaatccagagctgtctccattaggccaggctctcaccccagctccaaaccaacttctaaaaacttgtccaagagtcctcctcttctttagaattggtaatcttggcaattaaattcagcgtagaaacactctcctgaacataatcagcatgctggttcttccttttctgttgccttgctcttcctaacagctcctcctttcgtctttgcaggctgcttctctgtcacaggaactcagggctcagtgctgtacttcatctccaaagtgtccctaaagcgcccatctgatcccatggctaactactccccaaattttctcctggactgaccttactgaatttagatttgtacatccaatacctgcttaacatatccactttgatgctcagtgggcacctcacacttgatctgtcaaacactgaatttctgtctctgttatgcacatacccaaactttccccaccatgtatttccccatctcaataaactgcaatagctcaagccaaaagcctaagattcagacctgaattctttcctttcctctctctcaaatgcaattcaacaattttcttaccttttattttttgttttggaatgaaggcacatataactgagctagtaataatgcttgattcataatacaccaccgatgttccatgcataactctcttattcatttgtccatgcatttattttgtttttgaatttttttaaaggggggcaaggtctacgttgcccaggttggaatatagtagctattcacaggtgaaatcatagcacactatagccttgaactggcctcaaggatcttcctatctcagactcccaagtagctgggactataagcacgcaccactacacccagctcatgtacttacttttaatgacaaatgaaccaccccaaaacccaccacctaacccagggactaaaacattaccagtgacttactcatagatttgctcctcctctacctctccagaggtaaccactatcttgaactttattactttttaaaagttttgtcacatatgtcaatgcctaaacagctgttcagttttagttgttcttgacttttataagaaaagtatcatgtcacatatagttttctcagaattgctttttcattctgagttattgtgctgcaagtagctggtattcattcattttgctgccatgtaataatcacccattctgtgaacacattacaccttcctaaaaatagacattttaatttattccagaacattcttatatgtgtgatctgggggacctgtgcaagcatttctcaagtatatactgaaaagtgaaattgctgacccatgggtatactttttttttttttttaaggtatgatcttactctgtcacccaaggtaagagtgcagtggcacaatcatgattcactgcagcctcaacctcctgggcttaagcaatccttccacctcagcttcccaagtagctgggaccacaggcatgcaccaccatgcccagctaattcaaaaaaatctttttgtgcagatgtggtctccctatgttgctcaagctggtcttgaactcttgggctcaagtgatcctcctaccttggcctcccaaagccaagaggcatgagccactgggcctggcccaacttttctagtgaatggtttttcacagtggatataccaattgatacccccatcagcaatatgtgagtgatcctaatgactaaaaccctctccaaaacttgactttgtgtttcttcattttcaccaatcgaatgaatttgaacatgtcattgtcatcttgatttacgttttcctgattgagagatgaaaacctcttaatgtttattggcccacatgcacttctaattgtgtggaaggcctggttcagtcttttgcctgtttttctgtgacactgtccttttttgttggtttgtagaatttctgcatacattcttgatactaagctattactagttataaatgttgcagatattgcctcacagtttgtagtttagctttagttttttttttagagacaaggtctccctatgttgcccaagttggacttgaacccctgggctcaagcaatcctcccacctcatcctcccaagttcatggacacagtgtgtgtgtgtgtgtgtgtgtgtgtgtgtgtgtaaatggagtttccctatttttcccaggcccgtctcaaactcctgggctcaagcagctcaagtaatccttctgcctctgcctcccaaagtgctgggattacaggcatgagccacaatgcctaactactgatgcacgatttctaaattaagaatttataatataccataacttatattcttttatggttatcttttatggtttttttttttcctgcttccagtttaagaagttcttcctaaagggagtaggatcaggaagataatcacattttctaaatatgtttcaatcacattttaatctataattccacatatagtttctacatcaagtcgtcatcctgttgcattaattttaaagagcatgcttctagtgtataaggttgaaaagcattcttccccttatagattactaaagatttattattaatgggtatactgattttctttagtcttactttttatttatcctttttaagtcatcaacaaactttttctgagtatttgattacctttctttcaaaccgtacagtatctcctggatttgtttctctttttatttaggtactttctccaaaagtgattttagtttgtacggaaaatcttctgaagctttgatggtacatattcttattaatgccctcacattagaataactattttcagaacataaaattgtaggttcaaagtttttttcaggttcaatttcacattcttgagctaggcatggtactgatggttttcaccataacatacaccaatgtccttttgtctgtgggctcccatccagcctggtggctgaagtcatctacaggtaagattgaccaaacctctgaacaggactgaaaaaaatgttatcttcagaaaaccagccctcttgtacactgctgctgtgaatacaaattgattaacttttctggatggcaatctagcaatgcagatcaaacatttaaaaatacatatatatctcgacacaattttatctccaggcatccacatgaaagaactccacaatgttcagaagtgtacagataaggatactcgtcacagcattataatatgaaaaataaactgaaaaccacctcatctccaaacacaattaaattatgttaaaattctataaacagggattaggatgtgtaggtttacccaagggaaaatatatttaatgtttaggtttaaaaagcaaaaaaaaagcctactttttgtttcaaaaatatgcatatgtaagtagaaaatatctgaaagctgaaaggctactatccaaaaatattaacagcagctttctctaaacagaaactaaagcagtttctcttttctttttgcttttctatacttattacatgtctaccacaaacctctttgttataatttctccagttgagtcagttttacaatttggaatgcagagatcaagtggttctataatcagcatatacttcgcacgtaccattcattcaatccacacccctttaaacccctttgacacacgtcaaactcatttacatctatgtccctccaatgacaatatagtggtcaacacatataaaacatgaatacactatatcaagacactcaggaatacatctctgggataaaatctgactgccttctattatattttaatgaataaccaaaataaagggattctttcagttacagagagcagaataattaaaatagtaactttcaaactttgtagcagcagaagtatttcttcaaataaaatcttttttgaaacccaatatagaaaacagataaaaataaagccattctagaggtgggggccttggaaagtgagtactatccactcagacttctttcttgcctctcacaaggaaggaagctactgtgtagtttgaaaattactatttaatacattctgctaaccctaaatgccatgtcagagctagaagagaaaatgtacacacattcaatctaacatttatttatttcaggttttttttttttttggcaactataaattacattcactagtacacctggaattcttcatagtgtgttcaactaaagaataagcaaacacagcatagatcagtttaaaagaaatcatggtacttcttagagcaatttgcaaaaggggaaaaaagtcttaggctcactccttggaaataaatatcaagtaaccataaaaatattcagccatttttcagttattcggggagttcaggcatggtcccacgcagagcatcagagttcctctttgaaataacccagctttgccaatgacatctcttttctcaactgcataacctcccaaaacatctgatcaacatcctgctgtttcacgagtccctgctgaatgtatcgaatgtatgtaaaaaagttacatacagaagtgattttggtcctccgcattcaactgcagaagctttcacaaaccggataggttgtaatcccactggttcaatgcttagagtattgttttccacagcctccagaacagctgaagccaactcactttttgagaatgttaaacatggaaagatatcttcctggtagattttgtctaagaaaggacacgtcctgtccattgtgggctcatccttccacaatcggaattcattatacaaggataagtcagcctctttgcagtcttttacaattggctgtatcacactgaggtcctgatgactgccactcatagcactgcttgtgcttttatttcttgtatgcccctttttaaaaggtgtctttccacctggcaaaggctcctgcgtaggtgatgttggagaactggacaatacaagtgtcttcaatgcagctacttcagcttgaagtacatcaatttttccttgtgcttcttttagctgtttttctgctgttgcctgcttgatatttgcttctctcaccattttatgagcttcctcaaatagactagctgtgagttcttccaattcctgtccaagttgatctcgcacttttgaaagcctctcacattcttcatcttttaacttcagttccctctgagcttttgcgagttcttcttttaatcgttcatagcccttttctctaacttccaaaacagatgggcttcgtaaacgagacagactatcagtactcaacccaaaaatatcatcactgccatcgcaagcctctgttatagtagcaccctgtaaaaactctctctctgcattatagttgtcctttcttgtagttaatttagttaatccagctgtgactccagaggtagagcaaggggctgggtctgtaacatgaaagctgatactagatatttccgcacaatttaaacgtctgggggatgaatacacgggttgtgtaggaagttcagaaacatctaatgcatttgcctggataggtacagaggataaagctgaagggtgtggccggtagatgacacttggtgaggtagtctgctcttgagttcctgattcatacacaccaagaaggtccggagaagtaggtgaagcaaggtttacttcatggaagccttccaagggatcattagccatagcaaaagcctcatcataagataacctgagactccgcggccatatacaccttacgacgtgtgtgtgtgtggcgggagatgggaggggaggaatcctgtagaacccagatcccatcattccagcaactgccagagcgttcgagaatgtcatgtctgtacctgtcttct

SEQ ID NO: 15995 - RNA, 6610 nt, Homo sapiens
  source 1..6610: mol_type = other RNA
gctgggattacaggcatgagccatcgcacctggccagtttttttttttttttttttttctaagtgcaatgggaagccactcaaagggctttaagcagggaagtgacattatctgattttcgttttataaagatccctgcggctgccgtcagtgattgtaggagggcaggagtggatgcaaggacagcagacattagtgcaggagttcaggtgaaagatgataatagcttgggcagagtggtagcagtggacatggagggaggtagacagatttaagatgtctcggagacagctgatggaatttgctgataactggaatgggagtgacaatgacaaataaaggaacctagaataagccccagaattttgcttaagcaactgagagttcagccatggcagatctgttaagcacaaaagttaaacacaaatacaaattcatactgcattggactcttttaagcagtgtcttatagaaaaaacattttatctagggaaaaatgcaacaacaaaaaccactgaaaacaaaagcctatgaataaaagcagacccgttttagactggatgcacaaaacaaaaacacacaggattcttgtggtggcgatgggagtaagtgaagacgtaacaggttgcaagttattttaaggactaagacccaatgttcagaaaccaaatcttgttcttccagtgtggatgcttagtcaaagactgtaaattgtcttcaagctgagagagaccatgaagagagaggagtggccacctaactaaccttcccagtttttgggagccaaacctagaccagaatgtaggtctaagtgactcccaatccagagctgtctccattaggccaggctctcaccccagctccaaaccaacttctaaaaacttgtccaagagtcctcctcttctttagaattggtaatcttggcaattaaattcagcgtagaaacactctcctgaacataatcagcatgctggttcttccttttctgttgccttgctcttcctaacagctcctcctttcgtctttgcaggctgcttctctgtcacaggaactcagggctcagtgctgtacttcatctccaaagtgtccctaaagcgcccatctgatcccatggctaactactccccaaattttctcctggactgaccttactgaatttagatttgtacatccaatacctgcttaacatatccactttgatgctcagtgggcacctcacacttgatctgtcaaacactgaatttctgtctctgttatgcacatacccaaactttccccaccatgtatttccccatctcaataaactgcaatagctcaagccaaaagcctaagattcagacctgaattctttcctttcctctctctcaaatgcaattcaacaattttcttaccttttattttttgttttggaatgaaggcacatataactgagctagtaataatgcttgattcataatacaccaccgatgttccatgcataactctcttattcatttgtccatgcatttattttgtttttgaatttttttaaaggggggcaaggtctacgttgcccaggttggaatatagtagctattcacaggtgaaatcatagcacactatagccttgaactggcctcaaggatcttcctatctcagactcccaagtagctgggactataagcacgcaccactacacccagctcatgtacttacttttaatgacaaatgaaccaccccaaaacccaccacctaacccagggactaaaacattaccagtgacttactcatagatttgctcctcctctacctctccagaggtaaccactatcttgaactttattactttttaaaagttttgtcacatatgtcaatgcctaaacagctgttcagttttagttgttcttgacttttataagaaaagtatcatgtcacatatagttttctcagaattgctttttcattctgagttattgtgctgcaagtagctggtattcattcattttgctgccatgtaataatcacccattctgtgaacacattacaccttcctaaaaatagacattttaatttattccagaacattcttatatgtgtgatctgggggacctgtgcaagcatttctcaagtatatactgaaaagtgaaattgctgacccatgggtatactttttttttttttttaaggtatgatcttactctgtcacccaaggtaagagtgcagtggcacaatcatgattcactgcagcctcaacctcctgggcttaagcaatccttccacctcagcttcccaagtagctgggaccacaggcatgcaccaccatgcccagctaattcaaaaaaatctttttgtgcagatgtggtctccctatgttgctcaagctggtcttgaactcttgggctcaagtgatcctcctaccttggcctcccaaagccaagaggcatgagccactgggcctggcccaacttttctagtgaatggtttttcacagtggatataccaattgatacccccatcagcaatatgtgagtgatcctaatgactaaaaccctctccaaaacttgactttgtgtttcttcattttcaccaatcgaatgaatttgaacatgtcattgtcatcttgatttacgttttcctgattgagagatgaaaacctcttaatgtttattggcccacatgcacttctaattgtgtggaaggcctggttcagtcttttgcctgtttttctgtgacactgtccttttttgttggtttgtagaatttctgcatacattcttgatactaagctattactagttataaatgttgcagatattgcctcacagtttgtagtttagctttagttttttttttagagacaaggtctccctatgttgcccaagttggacttgaacccctgggctcaagcaatcctcccacctcatcctcccaagttcatggacacagtgtgtgtgtgtgtgtgtgtgtgtgtgtgtgtgtaaatggagtttccctatttttcccaggcccgtctcaaactcctgggctcaagcagctcaagtaatccttctgcctctgcctcccaaagtgctgggattacaggcatgagccacaatgcctaactactgatgcacgatttctaaattaagaatttataatataccataacttatattcttttatggttatcttttatggtttttttttttcctgcttccagtttaagaagttcttcctaaagggagtaggatcaggaagataatcacattttctaaatatgtttcaatcacattttaatctataattccacatatagtttctacatcaagtcgtcatcctgttgcattaattttaaagagcatgcttctagtgtataaggttgaaaagcattcttccccttatagattactaaagatttattattaatgggtatactgattttctttagtcttactttttatttatcctttttaagtcatcaacaaactttttctgagtatttgattacctttctttcaaaccgtacagtatctcctggatttgtttctctttttatttaggtactttctccaaaagtgattttagtttgtacggaaaatcttctgaagctttgatggtacatattcttattaatgccctcacattagaataactattttcagaacataaaattgtaggttcaaagtttttttcaggttcaatttcacattcttgagctaggcatggtactgatggttttcaccataacatacaccaatgtccttttgtctgtgggctcccatccagcctggtggctgaagtcatctacaggtaagattgaccaaacctctgaacaggactgaaaaaaatgttatcttcagaaaaccagccctcttgtacactgctgctgtgaatacaaattgattaacttttctggatggcaatctagcaatgcagatcaaacatttaaaaatacatatatatctcgacacaattttatctccaggcatccacatgaaagaactccacaatgttcagaagtgtacagataaggatactcgtcacagcattataatatgaaaaataaactgaaaaccacctcatctccaaacacaattaaattatgttaaaattctataaacagggattaggatgtgtaggtttacccaagggaaaatatatttaatgtttaggtttaaaaagcaaaaaaaaagcctactttttgtttcaaaaatatgcatatgtaagtagaaaatatctgaaagctgaaaggctactatccaaaaatattaacagcagctttctctaaacagaaactaaagcagtttctcttttctttttgcttttctatacttattacatgtctaccacaaacctctttgttataatttctccagttgagtcagttttacaatttggaatgcagagatcaagtggttctataatcagcatatacttcgcacgtaccattcattcaatccacacccctttaaacccctttgacacacgtcaaactcatttacatctatgtccctccaatgacaatatagtggtcaacacatataaaacatgaatacactatatcaagacactcaggaatacatctctgggataaaatctgactgccttctattatattttaatgaataaccaaaataaagggattctttcagttacagagagcagaataattaaaatagtaactttcaaactttgtagcagcagaagtatttcttcaaataaaatcttttttgaaacccaatatagaaaacagataaaaataaagccattctagaggtgggggccttggaaagtgagtactatccactcagacttctttcttgcctctcacaaggaaggaagctactgtgtagtttgaaaattactatttaatacattctgctaaccctaaatgccatgtcagagctagaagagaaaatgtacacacattcaatctaacatttatttatttcaggttttttttttttttggcaactataaattacattcactagtacacctggaattcttcatagtgtgttcaactaaagaataagcaaacacagcatagatcagtttaaaagaaatcatggtacttcttagagcaatttgcaaaaggggaaaaaagtcttaggctcactccttggaaataaatatcaagtaaccataaaaatattcagccatttttcagttattcggggagttcaggcatggtcccacgcagagcatcagagttcctctttgaaataacccagctttgccaatgacatctcttttctcaactgcataacctcccaaaacatctgatcaacatcctgctgtttcacgagtccctgctgaatgtatcgaatgtatgtaaaaaagttacatacagaagtgattttggtcctccgcattcaactgcagaagctttcacaaaccggataggttgtaatcccactggttcaatgcttagagtattgttttccacagcctccagaacagctgaagccaatttttgagaatgttaaacatggaaagatatcttcctggtagattttgtctaagaaaggacacgtcctgtccattgtgggctcatccttccacaatcggaattcattatacaaggataagtcagcctctttgcagtcttttacaattggctgtatcacactgaggtcctgatgactgccactcatagcactgcttgtgcttttatttcttgtatgcccctttttaaaaggtgtctttccacctggcaaaggctcctgcgtaggtgatgttggagaactggacaatacaagtgtcttcaatgcagctacttcagcttgaagtacatcaatttttccttgtgcttcttttagctgtttttctgctgttgcctgcttgatatttgcttctctcaccattttatgagcttcctcaaatagactagctgtgagttcttccaattcctgtccaagttgatctcgcacttttgaaagcctctcacattcttcatcttttaacttcagttccctctgagcttttgcgagttcttcttttaatcgttcatagcccttttctctaacttccaaaacagatgggcttcgtaaacgagacagactatcagtactcaacccaaaaatatcatcactgccatcgcaagcctctgttatagtagcaccctgtaaaaactctctctctgcattatagttgtcctttcttgtagttaatttagttaatccagctgtgactccagaggtagagcaaggggctgggtctgtaacatgaaagctgatactagatatttccgcacaatttaaacgtctgggggatgaatacacgggttgtgtaggaagttcagaaacatctaatgcatttgcctggataggtacagaggataaagctgaagggtgtggccggtagatgacacttggtgaggtagtctgctcttgagttcctgattcatacacaccaagaaggtccggagaagtaggtgaagcaaggtttacttcatggaagccttccaagggatcattagccatagcaaaagcctcatcataagataacctgagactccgcggccatatacaccttacgacgtgtgtgtgtgtggcgggagatgggaggggaggaatcctgtagaacccagatcccatcattccagcaactgccagagcgttcgagaatgtcatgtctgtacctgtcttct

SEQ ID NO: 15996 - RNA, 701 nt, Homo sapiens
  source 1..701: mol_type = other RNA
gctgggattacaggcatgagccatcgcacctggcccaggaatttctgtcttctaattccagagcaagggctcttgaccacttcgccaagctgccttgaagtgtcagtatgttttgtaagttgacacttgatgcttgtttttggtatttaaaatgatcagtactttgtttcacaagtcaggctaattttaggttgtttcttgcaaaatctgaaacttcataaaactttacaaagtcatattgactagacttacttttctctggatcccataattctgtatgtgttgctgatcccactacatatttatggaggaaagaagaaattgtatgccaggcaccatcataaagactttatgtgtagtacttcgtttcatcttcacagcaacctttctgagctgttttctgcatccataaaatgaaagtaatataatcacgtgccttccttggtttagtgaggatgttgtgaaattcagtagatgtgaacatgccagaaattgtgtgccacagtgcctggcatatagggtacctagggagggagtggctcaatgaatattattgaataaatgagaagtgagtaagttgttagaattatcattaccttatatgtgaataattgaaattaaattagagctatgtagatcaagagttttcaaatctgaattttgtctcaatctaaaaacttttctccatttgtatgttttta

SEQ ID NO: 15997 - RNA, 2263 nt, Homo sapiens
  source 1..2263: mol_type = other RNA
gctgggattacaggcatgagccatcgcgcccagctgaatggatgttttatatgaccaaagctcttaaagctttccctgcagctccatgagctatggaaagaagaatctagaaagaagcccatgtgtaaggtatcaggtttgatataaatgggggtcactagatcttattctcagaccctcccaggctgaaggaggcccaccctagtccagcatctggagagcaaagctgccggggcagcacagacactgccctctttacacctcgctaatgtccaggagtccgcacttgtatgggaccaactcccaagagtacctgagagttctccctgtctggccctgttccaagacataaagatcaggagaaactgatttgtgtgtggacaaaaatagagaagcaagaaaaattcaatgtaactaaagctacccaccacctgacagccatctagaatgtacctgagccctgtgccagccatgaccacctctgtcatctcagcctcactgtcctgacacccccactgctagctagatcagagagagatgcagagagggccgggccccagggctttgagtctctctcctaagtgcaatcgatgaagcaggaggaatccaggctctgcctgccctggcagcagggtgcctcttcctagtctgtaggaggagggtttccccgaagaggccgaggcagagggagaggaggggaagagtctgtcagagaagaaccacaggagaggttgaccacggcagccttgagctcaaagagggacctcaagtcctaggcacagtggggtttttagtcactcacaaggggattgcggtcatcttgttgactctgacccttgagtttcttcttaaagatggaaattgaagtggaaggcttgtaaaaaatgctccagatttcccccgaagtccctggttgatgacaatccctaaggtcccctgaagcaggaacacgatgggatttgaatgtgacgtgcagaagtatctttgctacaatggctgtgactgtgaggatgaggagagttgccagaccatagactgtccatcctgggacagtctgaggtgggtggctggggctggtggtgatgacatagaggactttggaggaccgggcagcgctgacactgaggttggcctgctccgtgatcacctcggccaccgtctggttgacagcgggcctctcctgtggcagttcttccttgacggcttggtataaaacagcaaatccctgggcctgattgatgcgatcagagaagaaatacaagatgacgaagtccagagagacgttgaaggacagaggtgggcggctcctcccgtggaagcgggctaggacacggtgggtgtagccatccagaagctccaccatgtccgccgagtccctgatgtcaaatagggggaagctgaagtggatgtgggaggcccccggaacccggatggtccagtagcagaccctccccgtggcataggtgtcggggaagtcaggggaatagaccacagaagacatggctgagtagttcccaccgcaggcgcccacgagagtatcaaagaggatgatcctgccatcgccaccacagggttgggtgtgatccccgaagcagacgctgttgcattcggtactggctgcctccccgtacttccagtaatcaggattgtttccacagaagcaagcatagcctgactccatcccagcaaacttgaacctctgactccgacaaaaactgatgcaagtttgtatggtgagtttgttggacgttttactggtgccagttagaggaggtgggtttccatgatccttgtagcagccaaggtttccaggcatctggcaagcaggtatctcacagtacttccagtagacaccatcctcgtgctctgccacatagcaccaggggctcacgtctccatctggatttctgcaatagttgtgctcacccaggcccccctccccgttggggtatttcagagtgttgtatggatgctggaaagtctcgttccaaaacagacatggcttcccgccttgtagtgctgtccagttctgtgttcccctataatccgcaccattggctgtgaaacactcgggtccggggccgaggccggggctaggcgcgggccgggccgccagcgtgagcgccgcggcggagagcagggcgaggcgggcggctggcggcgccatgggccgtcagtgcggggccccggggcgcggcccggggtaaagggggcagcgcggggagccgggggcggccatgggagcaggacgcggggcccgagt

SEQ ID NO: 15998 - RNA, 1903 nt, Homo sapiens
  source 1..1903: mol_type = other RNA
gctgggattacaggcatgagccatcgcgcccagctgaatggatgttttatatgaccaaagctcttaaagctttccctgcagctccatgagctatggaaagaagaatctagaaagaagcccatgtgtaaggtatcaggtttgatataaatgggggtcactagatcttattctcagaccctcccaggctgaaggaggcccaccctagtccagcatctggagagcaaagctgccggggcagcacagacactgccctctttacacctcgctaatgtccaggagtccgcacttgtatgggaccaactcccaagagtacctgagagttctccctgtctggccctgttccaagacataaagatcaggagaaactgatttgtgtgtggacaaaaatagagaagcaagaaaaattcaatgtaactaaagctacccaccacctgacagccatctagaatgtacctgagccctgtgccagccatgaccacctctgtcatctcagcctcactgtcctgacacccccactgctagctagatcagagagagatgcagagagggccgggccccagggctttgagtctctctcctaagtgcaatcgatgaagcaggaggaatccaggctctgcctgccctggcagcagggtgcctcttcctagtctgtaggaggagggtttccccgaagaggccgaggcagagggagaggaggggaagagtctgtcagagaagaaccacaggagaggttgaccacggcagccttgagctcaaagagggacctcaagtcctaggcacagtggggtttttagtcactcacaaggggattgcggtcatcttgttgactctgacccttgagtttcttcttaaagatggaaattgaagtggaaggcttgtaaaaaatgctccagatttcccccgaagtccctggttgatgacaatccctaaggtcccctgaagcaggaacacgatgggatttgaatgtgacgtgcagaagtatctttgctacaatggctgtgactgtgaggatgaggagagttgccagaccatagactgtccatcctgggacagtctgaggtgggtggctggggctggtggtgatgacatagaggactttggaggaccgggcagcgctgacactgaggttggcctgctccgtgatcacctcggccaccgtctggttgacagcgggcctctcctgtggcagttcttccttgacggcttggtataaaacagcaaatccctgggcctgattgatgcgatcagagaagaaatacaagatgacgaagtccagagagacgttgaaggacagaggtgggcggctcctcccgtggaagcgggctaggacacggtgggtgtagccatccagaagctccaccatgtccgccgagtccctgatgtcaaatagggggaagctgaagtggatgtgggaggcccccggaacccggatggtccagtagcagaccctccccgtggcataggtgtcggggaagtcaggggaatagaccacagaagacatggctgagtagttcccaccgcaggcgcccacgagagtctggcaagcaggtatctcacagtacttccagtagacaccatcctcgtgctctgccacatagcaccaggggctcacgtctccatctggatttctgcaatagttgtgctcacccaggcccccctccccgttggggtatttcagagtgttgtatggatgctggaaagtctcgttccaaaacagacatggcttcccgccttgtagtgctgtccagttctgtgttcccctataatccgcaccattggctgtgaaacactcgggtccggggccgaggccggggctaggcgcgggccgggccgccagcgtgagcgccgcggcggagagcagggcgaggcgggcggctggcggcgccatgggccgtcagtgcgg

SEQ ID NO: 15999 - RNA, 3641 nt, Homo sapiens
  source 1..3641: mol_type = other RNA
gctgggattacaggcatgagccatcgcgcccagctgaatggatgttttatatgaccaaagctcttaaagctttccctgcagctccatgagctatggaaagaagaatctagaaagaagcccatgtgtaaggtatcaggtttgatataaatgggggtcactagatcttattctcagaccctcccaggctgaaggaggcccaccctagtccagcatctggagagcaaagctgccggggcagcacagacactgccctctttacacctcgctaatgtccaggagtccgcacttgtatgggaccaactcccaagagtacctgagagttctccctgtctggccctgttccaagacataaagatcaggagaaactgatttgtgtgtggacaaaaatagagaagcaagaaaaattcaatgtaactaaagctacccaccacctgacagccatctagaatgtacctgagccctgtgccagccatgaccacctctgtcatctcagcctcactgtcctgacacccccactgctagctagatcagagagagatgcagagagggccgggccccagggctttgagtctctctcctaagtgcaatcgatgaagcaggaggaatccaggctctgcctgccctggcagcagggtgcctcttcctagtctgtaggaggagggtttccccgaagaggccgaggcagagggagaggaggggaagagtctgtcagagaagaaccacaggagaggttgaccacggcagccttgagctcaaagagggacctcaagtcctaggcacagtggggtttttagtcactcacaaggggattgcggtcatcttgttgactctgacccttgagtttcttcttaaagatggaaattgaagtggaaggcttgtaaaaaatgctccagatttcccccgaagtccctggttgatgacaatccctaaggtcccctgaagcaggaacacgatgggatttgaatgtgacgtgcagaagtatctttgctacaatggctgtgactgtgaggatgaggagagttgccagaccatagactgtccatccttcaactctgtggcttccagcccccatgggtggcgcccaggaattgctacctgggacagtctgaggtgggtggctggggctggtggtgatgacatagaggactttggaggaccgggcagcgctgacactgaggttggcctgctccgtgatcacctcggccaccgtctggttgacagcgggcctctcctgtggcagttcttccttgacggcttggtataaaacagcaaatccctgggcctgattgatgcgatcagagaagaaatacaagatgacgaagtccagagagacgttgaaggacagaggtgggcggctcctcccgtggaagcgggctaggacacggtgggtgtagccatccagaagctccaccatgtccgccgagtccctgatgtcaaatagggggaagctgaagtggatgtgggaggcccccggaacccggatggtccagtagcagaccctccccgtggcataggtgtcggggaagtcaggggaatagaccacagaagacatggctgagtagttcccaccgcaggcgcccacgagagtatcaaagaggatgatcctgccatcgccaccacagggttgggtgtgatccccgaagcagacgctgttgcattcggtactggctgcctccccgtacttccagtaatcaggattgtttccacagaagcaagcatagcctgactccatcccagcaaacttgaacctctgactccgacaaaaactgatgcaagtttgtatggtgagtttgttggacgttttactggtgccagttagaggaggtgggtttccatgatccttgtagcagccaaggtttccaggcactccgagttgttcttttaacagtaagttctgatccatgctctgcaggtcaagagcagttcagatttccctctgctcccatttgagttgtacttcaggtctgcctcctgcttgttgtagctctacacataacacaccaaggggcagagatctggtttccacacaatggcccaccattcagccagattctgctttgtccctaaacattcattccccctggctcctgctgggtctgttatattcagatatgaactttccaggaatctgatcatgtcacaggactttttctgtatgacaagttcaatactaatcatgaatagcaggcttcatgcagaggtttagtattattcatgaaaattgtgactccacatccagaaatagggcaaaagtggcctaaaataggatggctgtatctctgttaaatccaccaggcaattacaaacatctcttgctacaaactgtaaaacaggttttgctcaactatgttaatcagacacactagaagtacaatatgctgccagactcaatgtctgaggtccggcttgatggggagccctggtccccacagggtaaactgaagggttttccaaagaaccaaagccagacaccacccaccctctatccccagaaaccaggtactatagagctctcattcccaacttctacaaatctctctgcccagaccatctcaaggctagctttagagattttagagggttatcaaggggccacagaaaaactgaaataatatttaattttccttttttggaacaggaaagcatatccggtaaatattacaaattagaggcatactaagcggtttatagcattttgttataattctttcttctggaacctggtttcaatgaccacatgaatcagtccctattggcccagactgtattttagaaatgcaagtcaaagattatctttccaaataaaagtgcccagattgaaaccccctctttaccactcccaagagaatgacacaggctggtactaaaagactatctttgtgttgaacaaatggaccgaggaaaatctgctttcctctccctctgcttctttcttctttacataactagaggcaaatgagatgtttttcattttaaaaatttgattaagcagactgagcaaaagcccattcttctggtctttactgttttctaagtttggggactggatgaaggcacactcaggttggaaggatagtgaagctaagcaaaaggtgagtactaggtctgcagcactggtcaggggctgcctttccccctggaggcctcagcattcagatgctattccaggtatcagtgaaagggttgccagatcccatacacaagactcctgacctgagaggtgagaaagagggcaatgcaaagagcaggtttaaataataagaaaaaaataacccagataggatgttacgaattcactgtctttttcctcagctctaggcactgagctcttctggcatattttaaaatacattatatatactacattaatagactccttatagaagcagatcttgctttagtttctgtggttcaaaccttctgcaagacctttctacacacagtattttctttaccttgtttaaaagtatagtcatgtatctcttaggcaaggtttcgctctgagaactgcattgtcatataattttgttgttgtgtgaccatcatagagtgcacttgcacaaactgagatgtgatagtctactacacacctagtctataatgggatagcctgtcactcctaggctacaaacctgagcagc

SEQ ID NO: 16000 - RNA, 2231 nt, Homo sapiens
  source 1..2231: mol_type = other RNA
gctgggattacaggcatgagccatcgcgcccagctgaatggatgttttatatgaccaaagctcttaaagctttccctgcagctccatgagctatggaaagaagaatctagaaagaagcccatgtgtaaggtatcaggtttgatataaatgggggtcactagatcttattctcagaccctcccaggctgaaggaggcccaccctagtccagcatctggagagcaaagctgccggggcagcacagacactgccctctttacacctcgctaatgtccaggagtccgcacttgtatgggaccaactcccaagagtacctgagagttctccctgtctggccctgttccaagacataaagatcaggagaaactgatttgtgtgtggacaaaaatagagaagcaagaaaaattcaatgtaactaaagctacccaccacctgacagccatctagaatgtacctgagccctgtgccagccatgaccacctctgtcatctcagcctcactgtcctgacacccccactgctagctagatcagagagagatgcagagagggccgggccccagggctttgagtctctctcctaagtgcaatcgatgaagcaggaggaatccaggctctgcctgccctggcagcagggtgcctcttcctagtctgtaggaggagggtttccccgaagaggccgaggcagagggagaggaggggaagagtctgtcagagaagaaccacaggagaggttgaccacggcagccttgagctcaaagagggacctcaagtcctaggcacagtggggtttttagtcactcacaaggggattgcggtcatcttgttgactctgacccttgagtttcttcttaaagatggaaattgaagtggaaggcttgtaaaaaatgctccagatttcccccgaagtccctggttgatgacaatccctaaggtcccctgaagcaggaacacgatgggatttgaatgtgacgtgcagaagtatctttgctacaatggctgtgactgtgaggatgaggagagttgccagaccatagactgtccatccttcaactctgtggcttccagcccccatgggtggcgcccaggaattgctacctgggacagtctgaggtgggtggctggggctggtggtgatgacatagaggactttggaggaccgggcagcgctgacactgaggttggcctgctccgtgatcacctcggccaccgtctggttgacagcgggcctctcctgtggcagttcttccttgacggcttggtataaaacagcaaatccctgggcctgattgatgcgatcagagaagaaatacaagatgacgaagtccagagagacgttgaaggacagaggtgggcggctcctcccgtggaagcgggctaggacacggtgggtgtagccatccagaagctccaccatgtccgccgagtccctgatgtcaaatagggggaagctgaagtggatgtgggaggcccccggaacccggatggtccagtagcagaccctccccgtggcataggtgtcggggaagtcaggggaatagaccacagaagacatggctgagtagttcccaccgcaggcgcccacgagagtatcaaagaggatgatcctgccatcgccaccacagggttgggtgtgatccccgaagcagacgctgttgcattcggtactggctgcctccccgtacttccagtaatcaggattgtttccacagaagcaagcatagcctgactccatcccagcaaacttgaacctctgactccgacaaaaactgatgcaagtttgtatggtgagtttgttggacgttttactggtgccagttagaggaggtgggtttccatgatccttgtagcagccaaggtttccaggcatctggcaagcaggtatctcacagtacttccagtagacaccatcctcgtgctctgccacatagcaccaggggctcacgtctccatctggatttctgcaatagttgtgctcacccaggcccccctccccgttggggtatttcagagtgttgtatggatgctggaaagtctcgttccaaaacagacatggcttcccgccttgtagtgctgtccagttctgtgttcccctataatccgcaccattggctgtgaaacactcgggtccggggccgaggccggggctaggcgcgggccgggccgccagcgtgagcgccgcggcggagagcagggcgaggcgggcggctggcggcgccatgggccgtcagtgc

SEQ ID NO: 16001 - RNA, 2220 nt, Homo sapiens
  source 1..2220: mol_type = other RNA
gctgggattacaggcatgagccatcgcgcccagctgaatggatgttttatatgaccaaagctcttaaagctttccctgcagctccatgagctatggaaagaagaatctagaaagaagcccatgtgtaaggtatcaggtttgatataaatgggggtcactagatcttattctcagaccctcccaggctgaaggaggcccaccctagtccagcatctggagagcaaagctgccggggcagcacagacactgccctctttacacctcgctaatgtccaggagtccgcacttgtatgggaccaactcccaagagtacctgagagttctccctgtctggccctgttccaagacataaagatcaggagaaactgatttgtgtgtggacaaaaatagagaagcaagaaaaattcaatgtaactaaagctacccaccacctgacagccatctagaatgtacctgagccctgtgccagccatgaccacctctgtcatctcagcctcactgtcctgacacccccactgctagctagatcagagagagatgcagagagggccgggccccagggctttgagtctctctcctaagtgcaatcgatgaagcaggaggaatccaggctctgcctgccctggcagcagggtgcctcttcctagtctgtaggaggagggtttccccgaagaggccgaggcagagggagaggaggggaagagtctgtcagagaagaaccacaggagaggttgaccacggcagccttgagctcaaagagggacctcaagtcctaggcacagtggggtttttagtcactcacaaggggattgcggtcatcttgttgactctgacccttgagtttcttcttaaagatggaaattgaagtggaaggcttgtaaaaaatgctccagatttcccccgaagtccctggttgatgacaatccctaaggtcccctgaagcaggaacacgatgggatttgaatgtgacgtgcagaagtatctttgctacaatggctgtgactgtgaggatgaggagagttgccagaccatagactgtccatccttcaactctgtggcttccagcccccatgggtggcgcccaggaattgctacctgggacagtctgaggtgggtggctggggctggtggtgatgacatagaggactttggaggaccgggcagcgctgacactgaggttggcctgctccgtgatcacctcggccaccgtctggttgacagcgggcctctcctgtggcagttcttccttgacggcttggtataaaacagcaaatccctgggcctgattgatgcgatcagagaagaaatacaagatgacgaagtccagagagacgttgaaggacagaggtgggcggctcctcccgtggaagcgggctaggacacggtgggtgtagccatccagaagctccaccatgtccgccgagtccctgatgtcaaatagggggaagctgaagtggatgtgggaggcccccggaacccggatggtccagtagcagaccctccccgtggcataggtgtcggggaagtcaggggaatagaccacagaagacatggctgagtagttcccaccgcaggcgcccacgagagtatcaaagaggatgatcctgccatcgccaccacagggttgggtgtgatccccgaagcagacgctgttgcattcggtactggctgcctccccgtacttccagtaatcaggattgtttccacagaagcaagcatagcctgactccatcccagcaaatctggcaagcaggtatctcacagtacttccagtagacaccatcctcgtgctctgccacatagcaccaggggctcacgtctccatctggatttctgcaatagttgtgctcacccaggcccccctccccgttggggtatttcagagtgttgtatggatgctggaaagtctcgttccaaaacagacatggcttcccgccttgtagtgctgtccagttctgtgttcccctataatccgcaccattggctgtgaaacactctgagtcatagggaagttcaaagcggcccagcggagagagagggcacgtcccgtccgtctgggtacaaggtcgtcccaggaccctaacctgcctctagcagggcgaacaagtccatcccgttcctcgcgaggcagaagttataatgtccgccaagcgggtgcagccgaggactcgggaaaaggggctgagcgccggctcctcccgcctccgctctgctctgcgc

SEQ ID NO: 16002 - RNA, 1954 nt, Homo sapiens
  source 1..1954: mol_type = other RNA
gctgggattacaggcatgagccatcgcgcccagctgaatggatgttttatatgaccaaagctcttaaagctttccctgcagctccatgagctatggaaagaagaatctagaaagaagcccatgtgtaaggtatcaggtttgatataaatgggggtcactagatcttattctcagaccctcccaggctgaaggaggcccaccctagtccagcatctggagagcaaagctgccggggcagcacagacactgccctctttacacctcgctaatgtccaggagtccgcacttgtatgggaccaactcccaagagtacctgagagttctccctgtctggccctgttccaagacataaagatcaggagaaactgatttgtgtgtggacaaaaatagagaagcaagaaaaattcaatgtaactaaagctacccaccacctgacagccatctagaatgtacctgagccctgtgccagccatgaccacctctgtcatctcagcctcactgtcctgacacccccactgctagctagatcagagagagatgcagagagggccgggccccagggctttgagtctctctcctaagtgcaatcgatgaagcaggaggaatccaggctctgcctgccctggcagcagggtgcctcttcctagtctgtaggaggagggtttccccgaagaggccgaggcagagggagaggaggggaagagtctgtcagagaagaaccacaggagaggttgaccacggcagccttgagctcaaagagggacctcaagtcctaggcacagtggggtttttagtcactcacaaggggattgcggtcatcttgttgactctgacccttgagtttcttcttaaagatggaaattgaagtggaaggcttgtaaaaaatgctccagatttcccccgaagtccctggttgatgacaatccctaaggtcccctgaagcaggaacacgatgggatttgaatgtgacgtgcagaagtatctttgctacaatggctgtgactgtgaggatgaggagagttgccagaccatagactgtccatccttcaactctgtggcttccagcccccatgggtggcgcccaggaattgctacctgggacagtctgaggtgggtggctggggctggtggtgatgacatagaggactttggaggaccgggcagcgctgacactgaggttggcctgctccgtgatcacctcggccaccgtctggttgacagcgggcctctcctgtggcagttcttccttgacggcttggtataaaacagcaaatccctgggcctgattgatgcgatcagagaagaaatacaagatgacgaagtccagagagacgttgaaggacagaggtgggcggctcctcccgtggaagcgggctaggacacggtgggtgtagccatccagaagctccaccatgtccgccgagtccctgatgtcaaatagggggaagctgaagtggatgtgggaggcccccggaacccggatggtccagtagcagaccctccccgtggcataggtgtcggggaagtcaggggaatagaccacagaagacatggctgagtagttcccaccgcaggcgcccacgagagtctggcaagcaggtatctcacagtacttccagtagacaccatcctcgtgctctgccacatagcaccaggggctcacgtctccatctggatttctgcaatagttgtgctcacccaggcccccctccccgttggggtatttcagagtgttgtatggatgctggaaagtctcgttccaaaacagacatggcttcccgccttgtagtgctgtccagttctgtgttcccctataatccgcaccattggctgtgaaacactcgggtccggggccgaggccggggctaggcgcgggccgggccgccagcgtgagcgccgcggcggagagcagggcgaggcgggcggctggcggcgccatgggccgtcagtgcgg

SEQ ID NO: 16003 - RNA, 8841 nt, Homo sapiens
  source 1..8841: mol_type = other RNA
gctgggattacaggcatgagccatcgtgccaggcctgccatggcgtttgtaaactgtcatggcactggtgggagtgtctgttagcatgctaatgcattataattacagtataattacagcagtgaggacaaccagaggtcactttcattgccatcttggttttgaccggcttctttaccacatgctgttttattggcaaggtctttatgactgtatcttgtgctgacctcctatctcatcccatgacttggaatgcctaacctcctgggaatgcagcccagtaggtctcagccttattttacccagttccctattcaagatggagtcactctggttcaaacgcctctgacactcccaatttttgcaggtgaggaaatggaagccttgaaagattaggtggctcactctaagtaacatcatgtacctggcagggatttctataaagtcataagatgtcagagactatgcttaagaaatatttttactttgaaacactttaagcaaacagttaaaaagtacccaccacactaccctgtaaaaatcttaacattgtgatgcctctgcatcaatttttagaaaaaaacaaagaaaacacaactgaaggccccatgtaccctccccaaatccatcaggtctcctgccttaggaaggcagaatggtgacttgcacacatcgttccaatacatgattttatactcatttcatattatttgaatccacagaaaatagattactgtgcaaaacaataacactttctatatgtccacaaggcttacatgctagacactattctaagcattttacatgcattacttcattgaccacccccccacccacaatcaccctgtgagattgccactactatcccattttacagaaaaagtgaaaaacaagttgaagtaacgtgcccacaggtacacagtatgcttaactttacactaagggtaccttgtatgtagcttcaccaactttctcagcataatttttcatctatctgtgttgagacgtaactctttcatattcactttccaaggaccaaaaacaacccatttatttatccattcttctgctgatgaaatgcaggcttttcccaatcttgctacctaaacaatacttcagtgaagtcttaaaatcattctctgttcacatggcacttctctaggatgcatccaggagtagttgctgggtggttaagtgcacacaaccttccaagattttgcaaattgcctggcacaatatttctcacaatttctactcataaagcagtgtgaattatcgttgttccacgcacttacccacacttgggctttcaaaaatgtgccagctttctgagtgtgagatggtctgtattattttacatttcagtcagtcttggtcagcaggggtggggcagaccacactgaacaggtgacagaaagaccttcaaatacccactccagccatctggctctcctcaaccccaacttcagttcctccaagggagtgggggaaaggtgggaagggttggaaggaaactgaatgttctccaggccaggatgagatgcaagatgagacctggtgctcagggcaatcagaaactgtcaactgaagccaaacagctcagaaccacccacagccgggttcctaaccagcaggtgtgtgtttgtgggtggcttccagtcaacatttcaccccacagccccttaaaaaaaacccaaccctgactcagccaaactaaattcagcttcagattccttaacagaggtaattttgtgcaagatattttctgcatggcaaacagataaataagcacccaaccctggcttccagagtgcttggtctggctatggagatgggcataaccaaaaacacaaacatcacctgacataggaaccaagagaggtggggccacgggtttagaggcacaagggtcagacaaggtcaggccttgaagaatgaagagctgaactggcagagagaggggtgtggcactccaggtgaagggaggcagcacaaggcagaacactctggggggctggcatggggaagggacaggaaagccaaatccaacattgattctgccaaaatctttagtagttagcaccaagtagtcaggcttctactttttttcctttcagctaatctgaattcattaatatttatataattatagtacttatagaactaaaattatttgaaaactcaggttattggacaaataggttcagtataatcccaaatataaacagcttacttcaggataaaataatttctgttcttttggccgggcacagtggctcacacctgtaatcccagcattttgggaggccgaggcgggtggatcacgacgtcaggagatcgagaccatcctggagatcgagaccatcctggagatcgagaccatcctggctaacacagtgaaaccccgtctctactaaaaatataaaaaataacccaggcgtggtggcaggcacttgtagtcccagctactgaggaggctgaggcaggagaatggtgtgagcccaggaggcagagcttgcagtgagcggagatcgcgccactgcactctagcctgggtaacagagtgagactccgtatcaaaaaaaaaaaaaaattcagtttttcacttcattctttgcacattttaaaatttgattagaatgtttagaaataagcacatttcattctataaaaatgacaggtcaggcacagtggctcacgcctgtaatcccagcactttgggaggcagaggtgggtggattgcttgagcccaggagtttgagaccagcatgagcaacatgggaaaaaaaaataaaagttttgtctctacaaaaaaatataaaaaattagctggcagggtggcacacacctgtagccccagctactcgggaggctcagatgggacctgagcctgggaggtcaaggctgcagtaagctgtgatcctgccactgcactccaccctgggcaaccctgtctcaaaaaataaaaaagacagtaaaaatatccctatactggggcaggaactttacaaggtatcctgtggcaaagggagcagagatggggggaaaggggtgctaaaagtttgattggaaagggacttttccatggttacaacaccaactgacatggaagctgcacctctgagagggccctggtcctagaggtcaaccacctgatggagagccttggtaaaccaagccctctttcaccaatctcaggaatcaggtagcacagccaagcactctaacttcacacataaggaaattgatgcagaggttcattgacttgctcaagatcaatcctgccaagaaaaggcacaccatgcctggaacccagatctgatgactccaagacccttcctatgactctggcccccctgcccagccacttctagtgccagttttgggacagtgaagggacatcttcagtgccatgaacagctgctgccgtaggaaggcaagaggatggcagaaccaagatgaccaaaccttcctgaggacaaagctgaacaggcatcagaacaccaacaggagacttctgccccgcccccaccatcctgtgacaccaccacacaatatcagagccttcattttcacctgctcatggcaatccagagcaggtaagattattccatactctactgaaaaagacatcttccaggttggtttcttctcatttcaagaaatgaccagctccatgaacgggcccctatagtcaggacactgctctactattaaaacattttatcctttcattcataatctgacctcttcaataatcagaagcaatgattactcacatgctttagcaatatcactcctttgcctttaagtaattgattcttgctttttgcttcaacacaagtgggtgggccagtgagggagctcctcccagaacaggctgccttttctcctgagagcagcaggcacatgcacttgttccttcgggttgaatctgattgctagcaccagatctcatacatggagaggggtatgtgaagctgagaggggcctgcagtgtgcaggggctagagacatgaacacaacaatggtaagcgtttatatctgctgaggccgaggatcctatagaaaattcagaaacggagtggggaggagtctgatttatgggaactggcagcaaggctaactgcatgagaagcctttcacccttttactgagtccttggatctgtggttaacccttataaaatataattcagattcaaaccacatcactcctcaactcaaaattgtccaaaagctccctgcctccctctgagccagctcaagcccccgtaatgacccatgatgctcatatggccgggcctgtggcctccctggcccctctccttcccttccagctggctccctgcactccatcccaggggcttccttcctgaggacaccagtcaagacccaatctcctctgcctgcaactctccctagagagctacctgctacctccctggcttccttcacgtctttgctcacatttcaccttctcagttgaggccctccctgaccagactatctaaaatcacgactgatctcccaatccagcactccctctgctcttctctgattcactttgtccactacacacatcaccatccagaatactgcgtatcccatttgtttgtcatctgtaaagatccaagatggcaggattttcatctgttctggtccctgctgggtctctggcaaacacaccagcgcctggtgtatgggagtgctcagcacatttctgttaaacagatggaccgctgctgcctatgcaggcctgtgggatggggatggcaacagggtactggtagagatccacacgccaagcgcttgagcccagcatcctgctctcctccacctgccgctgagaccactctaaccccctagcagatatccaaaagccagccaggaaggctgaagccccagccagaactccccagggggcatttgggaaggctaggagttcttgatgctgctgcttttaaagtcaacagaataggcatggccacaggccaaacttgaagacaaatctaggatcccactggcccctttccagcagccatagcccatgatgccacagatattctgtccaaccacaaagggcagtggtctctctcttcagagttgtggaaggagacctgaataggggagccgcaggctatggtgcagaggccactcctaggggccggagtctccagaagggctccaaaggacatggtgctgcacttccccagcgtcacatcctagcaggcaggctggggactccccgagctttcaaatccttgggattctgtcactagcttccaaaacagaaagggctgggccctttatcaaagttactccacaatgcctataattaagggttctctagcaggggactgagaacccacccccactgtcactgtcaggtcccaggctaatctctaatatggtttttcatatgccgagccaggttcgaagaccacctgaaggtctttccacacttgctgcatttgaagggcctctctcgagtatgaaatctcttgtggctaatgagttgtgaactcttgttaaaagttttcccacatatgctgcatttgtggcactttttcccaatgcttatgtcctggagtccagtgagcctggagctctggctgcaagcttctttgcagtcttcgaggggcatctcttcacttggttttagcttctgtaatctcaactttgtgtcctgagaggaagaccgtgcaggcgggctacgttcagcctgtgctgctctggtgtgtttcctctggtgactggaaagggtatgtctcccaatgaactctttcccacaccactgacatttgaaaggtctctctgtagagtggatcctctgatggttaacaaggcgatagtttctatcataagatttcccacatagattacatttatagcgcttctctccactgtgtattcccttatgatctaaaagggttcttttacgtgtaaaggttttcccacattcttgacaccaaaaacgtttctcaccagtgaggatttttggctccacatttggagtcttttcactttcatggcaatcatactgtttttgaagagagtgaatcctctgatgtcggtagagattggaactccatctgaaggctttcccacactccctgcacttatatggcttctctccagtgtgaactctctgatggatgaggaggaatgagtgattgcggaaggccttgccacactggctgcatttgtagggctcctctttggagtgactgctctgaggaacctggaacactgtgtcctgactaaaagatggcccgccctcaggttttcttttcatggcatgcttcttcttatgaacaataaaggctgacctataggcaaagtccttcccacaatcgctacactggtaaggtttctcacctgtgtgaattctctggtggtcaacgagagttttctttctagtaaaagttttcccacactgctgacacagaaatgttttctccacagcgggagcaccctggggctgactgcagtcaggagattgcctgaagccttcacgacattcatcttgtttgtagaatttttcctcctcatgcaacctcatatgacgagtaaagtttgatctccatctaaaggttttcctacatttggtacatttatagggcttctcctgggtgtgaatcctttgatgttcaagaacatatgacttacagtggaaggatttcctgcactggctgcagtcaaagagtttctccccactttggtctcccaaatgatgatcaaaccctgagctgtaggtgagagctgccctatactgattcaattcaagaaatttcttcttagcatgggtttctcggtgcagacggtaggctgacaggcgtcggaaagctttctcacataaatcgcatttataaggcttcactccagtgtgaattttctcatgccgcgcacagttggaactccaccggaaggctttcccacacaccctacatttaaatgctttctcttgagtgtgaagtctctgatgatacgcaagatgggagctatgactgaaagtccttccacagtcactgcacttaaatgacactcccactgtgtgaagactctgcccacgttggtgatgagagctaaggctgaagtcttttccacacacgtcctttttgttccctttcagtccactatgaattctctgatgtaggctgaagcccccaatcatgtgtctgagccccttcccatatttcttgtagtcatagtggtgtgaactcattctgaagtgtttgccacagccatgtttaagggattcctttcttccagaaactctcaaatatgtaacatgttttaagtcaagactattacttcctgatacttcagagtcttttcctgtcctgtgactgaaattggtctcttctttcttaactcttacttgtatgggattttcacattgatccttctgcctgctcttctgttgaaaagattctctgagcccaattccctcagaaacacttgtcgcaggacatcctgatgacacagctaaggtttctgcttcttccaaaggttcctgatttaagatgaatttgtttgttttactctggaggtcatctcctgtaggagcagcaactggattccccttaggctgagctgcctgcatgttcaggccccatggctcccttgcttccaaccaggagatcagagcaggtttggtgaatggtcccaccagggaagccatgttcctataattctccagcatcacatccctgtacaggttcctctgagcagagtccagccacccccactcgtcctgggagaaggtcacctccacatccttgaaagtcatggtctcctggagctgggctgtcagggacctggttggtgttacctggtctcccgggcacccctctctcgggaaaagggcaggcatctgggcagcaggagtatcggattgcccagccaggaagtcacgtgcttctatttcatagggaggctccaggtggtcccccagagcagagctgctcctgagaggtgaagcaagggaccatatctgtgcagatcgcagggctcctgtacccatccaatgcacatctgggctctgggcagggcccgggtccctccaggatgtcccatcaaggtccctctgcagctcctccagcaaggccacagcctcctcgccactctcagggttatgaagctgcacccaaacccggagctccccaggcaggatgctcaggaactgttccagcaccagcagctctaggatctgtgccttggagagaacgtcaggcctcagccaccagcgacagagttcccggagccggctcagagtttctaggggccctgaagactcatggtagcgaagctgtctgaagagctggcggaacagctcctggccagggcggttgagagtctgtggcctggcagcctgcactggagtatagctttcatcctcttcttccttctttactgtctgaagccgccctcgctccctcgaagactgggcctgagctggataggcagcatgccacctgcctggaggcatcactcctgttcagggactaaccagaagagtgcgaaccaagtccaccttagacgtgggtcctcagaagtatcttctcagcagtcaacaatgccaacatttgctgggacatcagaagtcatcagcaagtgactgaaattaccagcatttctgtagtcccagctactcgggaggctgaggcagaagaatcacttgaacccaggaggcggaggctgcagtgagccgagatcatgccattgcactccagccttgcgaaagagcgagactccaccgactcccgccgccgagcgacaatcggtccacccgccgccaccgcagccgcccgtcccgcgcctacctcccggcggctcc

SEQ ID NO: 16004 - RNA, 8684 nt, Homo sapiens
  source 1..8684: mol_type = other RNA
gctgggattacaggcatgagccatcgtgccaggcctgccatggcgtttgtaaactgtcatggcactggtgggagtgtctgttagcatgctaatgcattataattacagtataattacagcagtgaggacaaccagaggtcactttcattgccatcttggttttgaccggcttctttaccacatgctgttttattggcaaggtctttatgactgtatcttgtgctgacctcctatctcatcccatgacttggaatgcctaacctcctgggaatgcagcccagtaggtctcagccttattttacccagttccctattcaagatggagtcactctggttcaaacgcctctgacactcccaatttttgcaggtgaggaaatggaagccttgaaagattaggtggctcactctaagtaacatcatgtacctggcagggatttctataaagtcataagatgtcagagactatgcttaagaaatatttttactttgaaacactttaagcaaacagttaaaaagtacccaccacactaccctgtaaaaatcttaacattgtgatgcctctgcatcaatttttagaaaaaaacaaagaaaacacaactgaaggccccatgtaccctccccaaatccatcaggtctcctgccttaggaaggcagaatggtgacttgcacacatcgttccaatacatgattttatactcatttcatattatttgaatccacagaaaatagattactgtgcaaaacaataacactttctatatgtccacaaggcttacatgctagacactattctaagcattttacatgcattacttcattgaccacccccccacccacaatcaccctgtgagattgccactactatcccattttacagaaaaagtgaaaaacaagttgaagtaacgtgcccacaggtacacagtatgcttaactttacactaagggtaccttgtatgtagcttcaccaactttctcagcataatttttcatctatctgtgttgagacgtaactctttcatattcactttccaaggaccaaaaacaacccatttatttatccattcttctgctgatgaaatgcaggcttttcccaatcttgctacctaaacaatacttcagtgaagtcttaaaatcattctctgttcacatggcacttctctaggatgcatccaggagtagttgctgggtggttaagtgcacacaaccttccaagattttgcaaattgcctggcacaatatttctcacaatttctactcataaagcagtgtgaattatcgttgttccacgcacttacccacacttgggctttcaaaaatgtgccagctttctgagtgtgagatggtctgtattattttacatttcagtcagtcttggtcagcaggggtggggcagaccacactgaacaggtgacagaaagaccttcaaatacccactccagccatctggctctcctcaaccccaacttcagttcctccaagggagtgggggaaaggtgggaagggttggaaggaaactgaatgttctccaggccaggatgagatgcaagatgagacctggtgctcagggcaatcagaaactgtcaactgaagccaaacagctcagaaccacccacagccgggttcctaaccagcaggtgtgtgtttgtgggtggcttccagtcaacatttcaccccacagccccttaaaaaaaacccaaccctgactcagccaaactaaattcagcttcagattccttaacagaggtaattttgtgcaagatattttctgcatggcaaacagataaataagcacccaaccctggcttccagagtgcttggtctggctatggagatgggcataaccaaaaacacaaacatcacctgacataggaaccaagagaggtggggccacgggtttagaggcacaagggtcagacaaggtcaggccttgaagaatgaagagctgaactggcagagagaggggtgtggcactccaggtgaagggaggcagcacaaggcagaacactctggggggctggcatggggaagggacaggaaagccaaatccaacattgattctgccaaaatctttagtagttagcaccaagtagtcaggcttctactttttttcctttcagctaatctgaattcattaatatttatataattatagtacttatagaactaaaattatttgaaaactcaggttattggacaaataggttcagtataatcccaaatataaacagcttacttcaggataaaataatttctgttcttttggccgggcacagtggctcacacctgtaatcccagcattttgggaggccgaggcgggtggatcacgacgtcaggagatcgagaccatcctggagatcgagaccatcctggagatcgagaccatcctggctaacacagtgaaaccccgtctctactaaaaatataaaaaataacccaggcgtggtggcaggcacttgtagtcccagctactgaggaggctgaggcaggagaatggtgtgagcccaggaggcagagcttgcagtgagcggagatcgcgccactgcactctagcctgggtaacagagtgagactccgtatcaaaaaaaaaaaaaaattcagtttttcacttcattctttgcacattttaaaatttgattagaatgtttagaaataagcacatttcattctataaaaatgacaggtcaggcacagtggctcacgcctgtaatcccagcactttgggaggcagaggtgggtggattgcttgagcccaggagtttgagaccagcatgagcaacatgggaaaaaaaaataaaagttttgtctctacaaaaaaatataaaaaattagctggcagggtggcacacacctgtagccccagctactcgggaggctcagatgggacctgagcctgggaggtcaaggctgcagtaagctgtgatcctgccactgcactccaccctgggcaaccctgtctcaaaaaataaaaaagacagtaaaaatatccctatactggggcaggaactttacaaggtatcctgtggcaaagggagcagagatggggggaaaggggtgctaaaagtttgattggaaagggacttttccatggttacaacaccaactgacatggaagctgcacctctgagagggccctggtcctagaggtcaaccacctgatggagagccttggtaaaccaagccctctttcaccaatctcaggaatcaggtagcacagccaagcactctaacttcacacataaggaaattgatgcagaggttcattgacttgctcaagatcaatcctgccaagaaaaggcacaccatgcctggaacccagatctgatgactccaagacccttcctatgactctggcccccctgcccagccacttctagtgccagttttgggacagtgaagggacatcttcagtgccatgaacagctgctgccgtaggaaggcaagaggatggcagaaccaagatgaccaaaccttcctgaggacaaagctgaacaggcatcagaacaccaacaggagacttctgccccgcccccaccatcctgtgacaccaccacacaatatcagagccttcattttcacctgctcatggcaatccagagcaggtaagattattccatactctactgaaaaagacatcttccaggttggtttcttctcatttcaagaaatgaccagctccatgaacgggcccctatagtcaggacactgctctactattaaaacattttatcctttcattcataatctgacctcttcaataatcagaagcaatgattactcacatgctttagcaatatcactcctttgcctttaagtaattgattcttgctttttgcttcaacacaagtgggtgggccagtgagggagctcctcccagaacaggctgccttttctcctgagagcagcaggcacatgcacttgttccttcgggttgaatctgattgctagcaccagatctcatacatggagaggggtatgtgaagctgagaggggcctgcagtgtgcaggggctagagacatgaacacaacaatggtaagcgtttatatctgctgaggccgaggatcctatagaaaattcagaaacggagtggggaggagtctgatttatgggaactggcagcaaggctaactgcatgagaagcctttcacccttttactgagtccttggatctgtggttaacccttataaaatataattcagattcaaaccacatcactcctcaactcaaaattgtccaaaagctccctgcctccctctgagccagctcaagcccccgtaatgacccatgatgctcatatggccgggcctgtggcctccctggcccctctccttcccttccagctggctccctgcactccatcccaggggcttccttcctgaggacaccagtcaagacccaatctcctctgcctgcaactctccctagagagctacctgctacctccctggcttccttcacgtctttgctcacatttcaccttctcagttgaggccctccctgaccagactatctaaaatcacgactgatctcccaatccagcactccctctgctcttctctgattcactttgtccactacacacatcaccatccagaatactgcgtatcccatttgtttgtcatctgtaaagatccaagatggcaggattttcatctgttctggtccctgctgggtctctggcaaacacaccagcgcctggtgtatgggagtgctcagcacatttctgttaaacagatggaccgctgctgcctatgcaggcctgtgggatggggatggcaacagggtactggtagagatccacacgccaagcgcttgagcccagcatcctgctctcctccacctgccgctgagaccactctaaccccctagcagatatccaaaagccagccaggaaggctgaagccccagccagaactccccagggggcatttgggaaggctaggagttcttgatgctgctgcttttaaagtcaacagaataggcatggccacaggccaaacttgaagacaaatctaggatcccactggcccctttccagcagccatagcccatgatgccacagatattctgtccaaccacaaagggcagtggtctctctcttcagagttgtggaaggagacctgaataggggagccgcaggctatggtgcagaggccactcctaggggccggagtctccagaagggctccaaaggacatggtgctgcacttccccagcgtcacatcctagcaggcaggctggggactccccgagctttcaaatccttgggattctgtcactagcttccaaaacagaaagggctgggccctttatcaaagttactccacaatgcctataattaagggttctctagcaggggactgagaacccacccccactgtcactgtcaggtcccaggctaatctctaatatggtttttcatatgccgagccaggttcgaagaccacctgaaggtctttccacacttgctgcatttgaagggcctctctcgagtatgaaatctcttgtggctaatgagttgtgaactcttgttaaaagttttcccacatatgctgcatttgtggcactttttcccaatgcttatgtcctggagtccagtgagcctggagctctggctgcaagcttctttgcagtcttcgaggggcatctcttcacttggttttagcttctgtaatctcaactttgtgtcctgagaggaagaccgtgcaggcgggctacgttcagcctgtgctgctctggtgtgtttcctctggtgactggaaagggtatgtctcccaatgaactctttcccacaccactgacatttgaaaggtctctctgtagagtggatcctctgatggttaacaaggcgatagtttctatcataagatttcccacatagattacatttatagcgcttctctccactgtgtattcccttatgatctaaaagggttcttttacgtgtaaaggttttcccacattcttgacaccaaaaacgtttctcaccagtgaggatttttggctccacatttggagtcttttcactttcatggcaatcatactgtttttgaagagagtgaatcctctgatgtcggtagagattggaactccatctgaaggctttcccacactccctgcacttatatggcttctctccagtgtgaactctctgatggatgaggaggaatgagtgattgcggaaggccttgccacactggctgcatttgtagggctcctctttggagtgactgctctgaggaacctggaacactgtgtcctgactaaaagatggcccgccctcaggttttcttttcatggcatgcttcttcttatgaacaataaaggctgacctataggcaaagtccttcccacaatcgctacactggtaaggtttctcacctgtgtgaattctctggtggtcaacgagagttttctttctagtaaaagttttcccacactgctgacacagaaatgttttctccacagcgggagcaccctggggctgactgcagtcaggagattgcctgaagccttcacgacattcatcttgtttgtagaatttttcctcctcatgcaacctcatatgacgagtaaagtttgatctccatctaaaggttttcctacatttggtacatttatagggcttctcctgggtgtgaatcctttgatgttcaagaacatatgacttacagtggaaggatttcctgcactggctgcagtcaaagagtttctccccactttggtctcccaaatgatgatcaaaccctgagctgtaggtgagagctgccctatactgattcaattcaagaaatttcttcttagcatgggtttctcggtgcagacggtaggctgacaggcgtcggaaagctttctcacataaatcgcatttataaggcttcactccagtgtgaattttctcatgccgcgcacagttggaactccaccggaaggctttcccacacaccctacatttaaatgctttctcttgagtgtgaagtctctgatgatacgcaagatgggagctatgactgaaagtccttccacagtcactgcacttaaatgacactcccactgtgtgaagactctgcccacgttggtgatgagagctaaggctgaagtcttttccacacacgtcctttttgttccctttcagtccactatgaattctctgatgtaggctgaagcccccaatcatgtgtctgagccccttcccatatttcttgtagtcatagtggtgtgaactcattctgaagtgtttgccacagccatgtttaagggattcctttcttccagaaactctcaaatatgtaacatgttttaagtcaagactattacttcctgatacttcagagtcttttcctgtcctgtgactgaaattggtctcttctttcttaactcttacttgtatgggattttcacattgatccttctgcctgctcttctgttgaaaagattctctgagcccaattccctcagaaacacttgtcgcaggacatcctgatgacacagctaaggtttctgcttcttccaaaggttcctgatttaagatgaatttgtttgttttactctggaggtcatctcctgtaggagcagcaactggattccccttaggctgagctgcctgcatgttcaggccccatggctcccttgcttccaaccaggagatcagagcaggtttggtgaatggtcccaccagggaagccatgttcctataattctccagcatcacatccctgtacaggttcctctgagcagagtccagccacccccactcgtcctgggagaaggtcacctccacatccttgaaagtcatggtctcctggtctcccgggcacccctctctcgggaaaagggcaggcatctgggcagcaggagtatcggattgcccagccaggaagtcacgtgcttctatttcatagggaggctccaggtggtcccccagagcagagctgctcctgagaggtgaagcaagggaccatatctgtgcagatcgcagggctcctgtacccatccaatgcacatctgggctctgggcagggcccgggtccctccaggatgtcccatcaaggtccctctgcagctcctccagcaaggccacagcctcctcgccactctcagggttatgaagctgcacccaaacccggagctccccaggcaggatgctcaggaactgttccagcaccagcagctctaggatctgtgccttggagagaacgtcaggcctcagccaccagcgacagagttcccggagccggctcagagtttctaggggccctgaagactcatggtagcgaagctgtctgaagagctggcggaacagctcctggccagggcggttgagagtctgtggcctggcagcctgcactggagtatagctttcatcctcttcttccttctttactgtctgaagccgccctcgctccctcgaagactgggcctgagctggataggcagcatgccacctgcctggaggcatcactcctgttcagggactaaccagaagagtgcgaaccaagtccaccttagacgtgggtcctcagaagtatcttctcagcagtcaacaatgccaacatttgctgggacatcagaagtcatcagcaagtgactgaaattaccagcatttcgactcccgccgccgagcgacaatcggtccacccgccgccaccgcagccgcccgtcccgcgcctacctcccggcggctcc

SEQ ID NO: 16005 - RNA, 2880 nt, Homo sapiens
  source 1..2880: mol_type = other RNA
gctgggattacaggcatgagccatcgtgcccagccactctcactttaatactatgaaaaatgctacttagatttttttctatactgcctacattccaagttattaaagtttaaaaccgtatgaaagcatttatgaagattctgaattgtatttctcattaaaagaaaagaaatgtgagtcatgtcccgaggcttatgtagaggagaaagcagaaggccattgtcagtcattttgaaagttaaaactcagcacttaatgtgaatttagatccatttaagagaggattcctcagttttatgggtttgtgctcctctgagcatcctcagggaagtgagaacacaagacttctgttcttctaagcaaaaatcattatcaaatgaatttattaaagagctatcccgagcaaattgcaattgtatgtatgtagctacataggcttccatgggaattgtaaatggctagctgagggcactttcaattgattcagagtaaaacaatctgaggcttgtaacaaatgtacaaaaaactaaaatcaatgagtaactctaataggaagaaactgtttgcattccttatgttacagtttgcttgtaaactgtatgtactttgtttcttttctcaacactgttttaaaactccagcattttcacctaaaagaaaacacaggctcttcataaatacctgtgaacaaataaatgaaatggtgactgaaggcgatttctgcagtagctttctctcagagataattatttttttttttgagacagagtctcgctctgtcgcccaggctggagtgcagtggcgcgatctcggctcactgcaagctccacctcctgggttcacgccactctcctgcctcagcctccagagtagctgggactacaggcgcccgccaccatgcccggctaattttttgtattttagtagagacgggctttcactgtgttagccaggatggtctcgatctcctgacctcatgatctgcccgcctcagcctcccaaagtgctgggattacaggcttgagccactgcgcccagctcaaagataatattttatcttgaagctagtgcatcgatttgtaaagctcatttaattttctacatactcaggatttgcatattgacttaaaatctgactttatcatccatgccgttatcaactagacaaaaaaatgtatcaagcacccacaggatgcacagatctatctctgaactggtgtagtggtattaatctgttctaagactagaattacatttttttttttaagaagctacagtccactgaaaaggaagtattatggtttttctgagaagaaaagttgctaaatactgcagcaaactcaggcttttcctgagaaaagccacaaacaaaatcatctctgaaattttttaagcaacaacttcctgaagcgtggaatttatggggccagtgagacactaaaatttcacaactctcacatacattatctatctaggactcagtgaagatgttcttcagatttttatttaagttaaattggtaaaatacaaaaagaaaatctggattgagtttcaaatcatcttaaatagcaatcctatgaacaattataactgcaatttcaaacactaagacttaaatatacaacttgatcatacaattatctcaaaacatatgatcaaaaactttggtcaagagcttctttcatgaattcttcaaggacagctatcacatttttggcttcaggcatttcttcatgttccactttaacaatcttcaaaagtatatctccactaccacagttctttaggaacatgtaacatttaaacaaagcataatgattcatttctgcctgtcggataaatctcttcaaattgtttgtgtcttgtatggcctttagtttaaagttctccagtacttgtcggaaaagaaaagggttacctcctttggcaccatttaaaaaagcttgcatccaatcctcacaaaaccggttacttcctgcattgcagaactgaggctgggagctgctgcaatcgatgaccacagacttatgctgctcctctgtcatggccatgcacaaagaagtcatggtgccttcatgaataagtccttgaagactggccacactcagaaacctgttaatgtctctctttgttttttcatctgattctttaacttcaacaggagtgtaactcaaagcagcatgtagcagaaaggtaagcttttcctgaaagagaagaacaaccctttggattgggcatacaacatcctcaaaccagctgctcagataggattttatgtgactctccaggccccttgcctcacaattcatgttatttttcagcccttgaatgtacttgtccaattcaagcctgaaaagctcaagtcctttttcagaccctcctaaaaaacagaccacatattctgaagggttacgttcagagtctatcgttactgtttcaggaagcagtttttcattttggaaaaggcagtaataacaaccaactcggtaacctggaatttttagctccacagatgcaacattacccagcccttcaaagactgcacctcttgaaagacgcttagcaatgaaactgcgcagctctggctccacttcggatggtagattagtatctgccaaggagaggctgaaatcatcaccagagggagtttctgcatttgtgccacttgggcttccgtcctcactgtcccctcgttgctgtgccaatctgcttccgcgatagctgtaaagacagtagtggctgctggacggcggctcgagtctccgctcctcggctgagcctccctcttcgctgctctctagttccttttcatctccatccatcgactcctgcaaagaggggagcattgcggcggcctctgagcggccctgtgtctccgcc

SEQ ID NO: 16006 - RNA, 5425 nt, Homo sapiens
  source 1..5425: mol_type = other RNA
gctgggattacaggcatgagccatcgtgcctggccacacctgagcttttctgaaacttttcaaaaggaagtctagttaagtcctcaaagcttcagtttcatatttaaagaaggaaatctctatcaaaggagaaaagggtatctatttcatgccagccataaaatactgcccataatcctgttccttttctaccaaggctagcagcagagtgagctcaccgggaggcaaggtgccctgattctgagctgccggactaagatgttctggactctgagctgccggagggtaagcccctcagccctgagctcactggcctttgccacccaagctgggggacagtgcctgtcattaactgtaaaggtccacactgtgattcctttgggacaccacattttgaactcccgtgctataccaagtcaccttctggctcagaatcaagaaccacgcggacagagacgtcctcagggctctgactctttcttggtggttttgctctttaaccacactgccaaccctcatcctctctccccactatgtagaacattcttcctcttattctctatggaaagcgtaattctttagaactcctaaaaacctgaaacccattatactttcaattagatggcaagaatggcaacctcgaccagatgggaaagtcagcaaacctggcgtcattcaggaataacctaaacttcactgtgtttaattctttttaaaaaatgttctgtactccaaaccgaaatggaaagtttagtttcttttgagttgttctactgagtagtcaggttcctcagaaaatccatctctgatgaaatagggcccagactaataaggtggtgctctctccaactgaatgtacattctatagcataaagccaaagtctctgtctagacccctttggttatttttctctaccagtgattctgcccatgctctgagagtgtcagctgcaaaggcctgtgggtacttcacgagaaagatggattataaagatcttcaagattgtagaaggtttaaaagtcattaatggttgaaacatggctataaaatgttggtcccacctgcagggtacttaaaaaacttgctcagatgataataagggcacgtgcagtagcagaagctgcgttcacctggcttggctgggttctcatggctcccagggcacaccgcctagcctctgggcgcatcttccctctcccagaatgagcaccacaaggcctacatgaaccagctgttagggaagggaaaggatgcaactctgggaacctctcgttgaaggccaaatgggtaattctcttgtcccaccatggaaattctatgaccaactcctcctccacatttcctggcactggctgaccatctttaatttttatgagttttgtatatagctgcttgagatacatgtgttttgaacaagaggaaagtgtgacagacagaaacacagccctgctggccccctcttgccacagtgaccctgggccgtgaaccacctggagctgtatgtgggacattcagaacacccagcagtttgtggagctctggacgcatctcacaggcaagttttacaagttgctgagagaggccattttaaggaaaatctacataattcttcccaacaggcctggtacccacaaaccctgcgagtcctgtcatgctatgacaagaataaatgtgtttgtagaggtagagatggtactgttcacctcccaacacaaggaagtggtcatgaaagtgggacaggtgagggcttggacctcatgacaagcccagtggccaaggggtcaggacagggcatgtcccatcacggtgcagggcagacaggagagcagccacagctcatccacacacagtgacagggaacaggacgcagaatcttaagtgaaggtgaacccaaaacaagaccacggggcttaatcaacacagctccaggccgtcagaggagcttggaagcaaactgcatgaaggccgagtggccttggcctcaccagggcgggtgatgggagcagtgtctgagcgcctgcgagctcctgtctacctacacaggacctgggccgccctcaggtgtgatggtgcgggacggggctgagggacagcacttcacggctctgccgcccaccggacggccccatcactgggccacagcctgccagtggaactcccctctgatttgcaccagcacctccgacaggccatagagaaaggggactccgaacgcaagcagctggcacatgaaaaaggagtccagagggttttgggccacttgttgcccgaatgaagaaatgttgctttggaggtgctggctcatgcccttggccttgtcacagaggccgagggagtgacgcgccacccagccaaacaaggaagtgaggctacctggggttctctcagtggagctggccacggcgttggcccgtccgtttgcatctgtggtggcgccatcctgcaggggtcctttggcctcctttccagacaggggagccactgccggtctcttcctttgtgcgtagccagagagtcgatagcagtagtgtggcttacagtagaatttaccatcctcgatgtcgtaggcgtaggccgagaggcgcagggtggtggcgcagtactcgcacttgaagcagctccggtggaagaacttgccctcggcactcagcctctccatcacgtagacccgcttctggcagaagtagcatgtgtcgctgcctcccaggttctgcgggaactccttcttcatggagcccagttccttcttgtctagaagggctttgggttgttctttcctttgaagctgattggctatctgctcagccaatgagctcactccgcccgtgtacatctttatatacttctgtcggagggagtcggaggagggagaggcggggcgggcagaggagcggagactaagagaaagctcccactggtcgacaaaaaatcgacgaggaggttcaggctctggcctctcatggtgggggctctgcttgccacggttgtcagcatcaagatccctgtatgtctgctggccgccatgtgcccgacagggaggtggagtagggggaggagacagggtgatcacttttttggggcaggtccgagaacactccttttcccgttgctgtctccgtatgccgatggactgtgcgggcgcattctcttcaaatttggccagcagctgggtcgccatgtacttcactttgttctggttcccaacggcaacgtccatcctcctgtctgtcagagtgctcaccagggtcggtctttctcctctgtggccccgaggagcttcctcctcctctgattgactggtctttctcctcttcccagcaccatccaagtccttttcctttttatccttgggagaacgcttccgagagatggtctggccaagtttgcttaggaaggagataggggatctggtgctggctatcaggactgctttctcctcggcatttaggtccaaggtgtcgctagaggggagggagtccttaaacatctcgtagaactgagtcaggtacatcaccatggacagcttatcaggctcccccacggaggccatttctttgcctgtcatgatgggagaaatgcccaattccttctcagcaatgtcaaaggccagttggttattcttctccacattttgctcatccaaagaatcaaaatctatcaggtcagggcggtatctatggataattgcacaaagggccaagccacttttccaggacatggtgagatctgtcacgtttacccctgcatagccatctgtctgcctctggcaccaacccagcagtttgcttgaacgagctacagactcattgcgagtcaatttgggggtggttcgggaattcaccaggctctccatttccaggtgaatatcttttgtttcgccagtatcatataaatggcgcacctggcttggccggaggaagttgacgttgatattgggataccgagtgacagggtcgatactgtactggctgaagttcttactcacattctcaggggtggtctgaggcagcaacctgtaaatactttccctctctgccagcacttccaaagggctcgttcctagagaccaacttcggaccatccaggcagagtccatagcagctagaaagccccgggctattcctgttcccattggccagaaaggctctaggaggctgtccccgaccagagccactagtaactggtgtccgttctgctcccgcaccaaggcggcgttctcggaggcatacatacaagtgaagtcaaacatggccacatcgggctgcccatagtgattgatggcaaaatccagagacggcagctgctgctgggtagagaagtctgccgcctccctggcatagctgagcagagcctcctggtccacgttttctcgggaaagcaggagctctgtgtcggcgtagtcatgtagtatcactcctttgtccagcaaactctgctttttggctgtcataacgaaatagtgtgtgtcatctttgtagtaaacgatgttctccaagtcaatacctgtggcttccctcagttcctggaaaaatttttggttgaatataaaagccacaccactgatctcttccactttagcttctgctgttgtatttcggttgataaaatttgccgtgatggcgatggccagtttgccacggaattctttccgacgaaacccttccaaggtgttcctccgaccatccccaccgatgatcacttcaaattcatactctgacacaggatgagtcttggggtgcaccagtgcccgccagcctatccgttcattctcttggtcctcaggaggctgtataagtccttggaattccacattgacgtggatttcaatgcctaggatcaaggctactttcaaaagtattagttggagctgacggatactgatatggtcgatggctccagcacagaacttgccatagaacttcttggcacccagacctcgtagatcatgtatggtgaatggccagagatgcaagacgttgttgcgggagaaggcatctcgtttctcaataacaaccaccttggcccccagtaaggataagtcgatggctgtacggagaccacaggggccagccccaatgatgagacacttggtgttagtgcacgcttttccctttttgtagtctttgtgactgccccgtttgtccaattttgcccagagggctttggctttccagtagttaagcttggacttgagcttgtgatagaaggagcggtagtcctttggctttagttccaggtggtcacagagctcctggaaagccttgagggttcccttgcaggtggtggcctggacaaaccggtcaaagaggacatgagctgggttcatggtctcatgcttcctctcctccatgctgcctcactctcagcactccccagagggggaggtgggatggctgtgggtccacctgacactgtcacgttaat

SEQ ID NO: 16007 - RNA, 2251 nt, Homo sapiens
  source 1..2251: mol_type = other RNA
gctgggattacaggcatgagccatcgtgcctggccagaaatgatgactttcttagcaactcttcctccactgctcctttaaatccaacttgaactcagtctcttcatggacaatttaagtctcaattgccttctgcctctgcctctccctttgcttggccctctcagactctcgcttctcatactctctgcgatattcttccctcttcagcctctcgtgctgatattcctcgtagctgtcatacctgggccgacggctgtagggcgatcttgaacgtgatctcacatacaagggagaatttcggtgcgtgcggtgtctgtagtggcttgactcatagtaatagcaggatcttgaagaggatctactgcctggagaccttgatcttgacctggaatatggtgatcgggaacacgacctgtgtcgagaaaaggaccttgaacgagagcgcatcctttggggtctttgagaaaataaggatttgggtggtgacacagaatctctacatggagagttaaaagaagaacaagaaggagacacattgaacaatgaataggattgcgtgccatcccaagggtagctcagtttatcactttcatcttcgctgtcatcaaacaggccatccatggctagtcctgaatttataaacataggtagtttggagaattgttcattactgaaatcactgtccctcagttcaccggtcttgtctgcttcgtcgtcaaaaacagcttgactgggatgaccgaagtgcttgttcagctcggctcggatttcctggtcttggagctgttttcttgtgctgcaaggagagacctgcttgcttgcctccaaagtctctctcaggtagcactggtctgaatctgtggaagaacaaatctgcccctgccaatcagaggagacatctttattttctagttgtctagagtcttggagctcctgtgatatattaatgagtatttctgttttggaattaattgactggcaatagtcatggtcaccaaacagccgcagactgggccgcttggtcttcctttcctcgtgtccaccagtgaggactgaggacttgctgagttgtgcatacaactcggattgctccggccctttcttggtggagttattgccttgtgtaccagaagactcactgtacctgggcttctttgatggtggtggcaccacagtcttgcaagaggacttcagctttggagaagccctaaaagggttatcttggttggctttatgaggaggagtggtgggtggagttaggcctgcagttccagagagttccacacttaaggtgcgttcaatagtcttgttctcaaatggggaacccttggggtcatttggtgactctggggtcagaggaagagataaagttgttggtttggcttgtaagtgttgtgactgcgactgtgtgtgggacttctttttggaggtgcatttgtctctgctgctgtttctgttctctgtgggtttggtgtgaggagggtcatcgtttgtggtcagatatttgagaagctccgagcagggacgtctttgtggcttttgctgttgacaaatactcttcgctttattgctccatgaattctcagtcttaacaattgcagggtttgttctgatcctgtgattgtgatttgcatggttctgggtactgagaccactgcattcattataacttagctgagtgttggctggtgccagtaagagcttcttaagtagagacggctcttctgcctcctggggtggaggggtgccgtcaggcatggaggaaggactagcctcattgtcagtggtcacgtctccatctgtcagcgcatcaaatgagggcaatccgtcttcatccacagggagactgtctagtgtctctgtgaggactgctagcaagtttgcctcattctcttcatctatcttctcaaatatgtttgaaggctcattgttgtactgattggatattatttctgattggtcactgcaccacttgagtccacccagaaagctgtctgtatccaagtcgttcacatctagttcagaaagatcaagttcaggaagatctgggcaaagaggctggtcttcaccaaccagagcagcacactgccagcctgcttctcgctgaagtacttttttccagtcttcttccagccttggggaggtctcatccattgctgatgctgcttgcacaaactggattcgccagcggctgttactctctctccttgcaagcttttaccaaagcagcagccagggcagtccaggg

SEQ ID NO: 16008 - RNA, 840 nt, Homo sapiens
  source 1..840: mol_type = other RNA
gctgggattacaggcatgagccatctgctgaactttcaattaatccttcagtctggtgatcccagttgcccagacccttacctccaggtgaagtcaaccaggtgcctccaaagcttgctctttcctcccctgggtatgtgtcagagggacagacacctttttcaatggtgatcctgtgacggagacctgagcgtctttggagagatgctggaacaggagaacgatgcttcacaattgctgctccagggatggaactgtggtccaagaacagatacttcacactccaccctaccccaccaggggcttctgtgtgcaaaatcacttcctacagggaggcaatgtgggcaggctgggaggtcggttgacttggatgattgttacgacttagccaatggtattaaatatacacgtctaacaggagtcccagaagaaggttactgagatgatcagacctgtcttgttgaagagacaactctggaggctaagtgcagcctcttgtagtctattcttgctgcatgttggagatctccaccagagaccgatgagatccaggttttccatcatctagcatctcccctctagaatggatttttcctcatctgcgtcacatcctgcaattcttaagggatttggtatggggatgtacaaaataagctagtcaacagggggcgggcaggtgggggcagggagaaaaggaaagtaaggaaaaggcaccaagttcagggctccttaaatccagctcccagatcttaccagaacaaatcgtcaaaactaatcttcttttttctttttctttgagacagagtcttgctctgtcacccaggctggagtgcagtggtg

SEQ ID NO: 16009 - RNA, 239 nt, Homo sapiens
  source 1..239: mol_type = other RNA
gctgggattacaggcatgagccatcttgcacagtctggtaatatttttgatgtgttgattctttccagtccagatgcataatctcatccctaaacattcctgctggtgtgattatgacatatcactttacccagcaccagagtgatttgatgctcctccctgggcccaggccacaaatgggattgtgacatatccctggacccagagaggtggtgtgacaattctactgccttggcact

SEQ ID NO: 16010 - RNA, 723 nt, Homo sapiens
  source 1..723: mol_type = other RNA
gctgggattacaggcatgagccatcttgcctggtccagatgctatattttgaattactgtactacaactgtctctgtacttggaacttgaatttgcttcttatctgtggacttcttggctttgatattggcctggcttattccacgtgcctatttgctgacttccatgatagtaccctcttcctgcccagaatcctgttcttcatcagccctcctaattgggcttctctctcttagatgtttttgcttcttctttgtttaggtataactcaggtccttggtaagatcacttcatcctttgggatttaaataaaattagcgtaaacactgtaactcttataatgtggaaaggtcaactgaagcctctaccaatatatctgtgaattaaatgaggcttatgttcttatggtcatatgttcctgaggactctcaaattcatttgtgccatcttctgcagtggttctattggccctaagctaatccatccatggaacctagtcccttttccttgatttcccgaaatacttttcttggaatgcattgcgtgtgtctatgtgtgtgtgtagaaattttatgaatttgaattggtaaaaagaattacatggaattaagttaaaagatgttagacttcctgttcctttctaaaagagttcattttcttgccaaaagggattttccagttgctaaatttttctgcaggccatcatgttgactgtgtccctga

SEQ ID NO: 16011 - RNA, 686 nt, Homo sapiens
  source 1..686: mol_type = other RNA
gctgggattacaggcatgagccatgacacccagccccaaactgctgataggttattttacaattataaatttatatcttgatgccacttacaaagttctaggcattggtgggtaacctggtttgctttcaaatggtcacaggacaaagaactgcctcctcacactcagaaacgtgtctatgaaggctatttccatttcacatttcagaacctgagagcctccaatacaaggaaacgagagttatttacaattttgatacacacacgcacctcaagatttaaggttctagattgaggagcctagaaatttgactctaaggcttgacctgctcacctagataaccaaattaatgaagctactggatacaacctcaatagagtacagagaaagcttctgcactccaaggactaaggtaacattacttcccaaatcagattaaaccaaagggggaacagaccttcacaagtcacggctatatagcaatttgggccaggcacagtgactcacacctcccagcatttggggaggaagagatgggtaaattgtttgagcccaggggttcaagaccagcctgcaatatagcaaaccccgtctctacaaaaaataccaaaaaattggccgggcatggtggctcacgcctgtaatcccagcactttgggaggccgaggcaggtggatcacctgagg

SEQ ID NO: 16012 - RNA, 7862 nt, Homo sapiens
  source 1..7862: mol_type = other RNA
gctgggattacaggcatgagccatgacacccggccatgtgaatttttttatccaaaaagaaccccgttttcctgcctacctacctcatccttaaaaaatttttaaatctatttccaaaggaaattatgtaaatttgtaaatagagcatttctgtagaatttttttggaaacgatgtctcactctgtcaccaaggatggagtgcaatggactccatggctcactgcaaccttgacctcctgggctcaagtgatcctcctgcctcagcctcctgagtggctgggaggcatgttttgaagggaatggctggactgcgggattttccacccgcttcgtacgcttcccgtctgttctcaatgagcacgaccgacttttcaatacaggggctgaatcagcctccacccgcttcatacacttgctgtctgttctcaatgagcatgactgactgaaacagaggggctaaatcaagctcagaagggaatgcacagattgggcgggtgcactgctgccctccacagactcaagtcagacaccggctccgtctctcctggactggaatgtaccgtgacctccaagggaagctctgtgtttctcattttaacctcggtcattttaaggcaggaactgtggccagttgggggtgtcatactcatttctggcaagggaacaaataaatttaaaaacctacaggagaaggccttgagccacacgctgagctgccctggggctccacatgctccccatactcatcacagagtgggctcagaccctgcacactcaggccccgaagatgtctcaagagggaattaaaagtcccgtcctggcccccgagaacccctcaggagcagcgactccatccctactccaacctgagtgggtgaaggcaagggaagcccacccagctcgcatcagcagtggacggacggagcccagcacccctgccagcattcagcccacaggcccggagaggggtctgccaacgcgtgtgacccgtctccagagagcagccacgagcctggcgacccacaccccacagcccggcccccagcacactccagaccccaggtgcagggtgagcctgctccaggctgaacagacgcagcccagggcctgggtggggaggcttttagtagttactggttggccgagcaacggccacttgggggaagacgatgaccagtgcggccttcacaagactgcccagaggtgccagcctgagggccctagcacgagatcacccgcagctgtgccagcaccaacacagccaagccatgcacagaccactcagcagccacgacggccccggctccgtgtgcatggagtggggccaggaaggggattaaaacacaaggcaagtccttaattctcagaaagaggagaatgataaaatgcccctcttaattttcctaagcattcagtgagtgcgcgtatgacgcaagaacacacagaggttctgcgtgtcacccatgaaaatgtgacagcacccgggaagacgtgggcagcacagacaaacccagcccaaccgagacaccacccagcaggaggcctggcgggggtgggacagctgcaaggcttgctaacaggcggtctgggggctgcggcagtgcggggtcacccaggaagccaagaagccagaccaggacacagacacatcccgggaggctctgcagccaccgcctggagtccccagaacctcgggggagctgcaaggtggcctgcgctgcccggaccctcccagcctccacctggaccaccagaaaataatctaagacagctatggttctgagatctctcaatctcggccctgccaactcccgccctgggaggctcttccagccagctgggagatgtccaccatgacccgcacctcagcacccctgcaaggacctcagcccagaacattctgaagcccaggccagccttgaggtggggcccaacgtggggaacccagggcctaaggtctgcagagatgggtgcccggtccatgaggcatttgcaaacagcaggcactgaggccgagcccaagcctctaaatcatgtaaatagcaaggggcaactttcagcaactttttcagcacgaggtttttttttaacgctgaaagtaaagctggtgactgtgagaaatacgttaaaagaggcggcggctgccaggaaagagccgctgccccatcaacacaggagctgcacggaattcccacagcggccagggtccacccaccctcaagggccttcccagtgacctcctaggaggccaaagactgaacacagaaatgtccctctctgcccccaaaggagatggcgcaaaggtgtcccacagcccagccaagcgcagtccccggaagcctgcccgtcaccaggtacgtccacagcacacctgaaactgtcccgggaggtccccaaagggtcttctgagagactgaaggccacagcggctgagacaccgcccctccccacagggaagagaagccccagggcccacctggggaggcggaggcctgcaggtctgactgatgggccgtagtctcctctggtctcaggctcccagcccccaacccatgtggacaccacaaatcctccaggccacaggtgtaagaacaccaggccctgatcagtggctgccgagacacctgagggcacggagccatgggaacgcaaccccacaacacgggatacaagcccgcccctgcccgcccctgccgctggcacccaagctgccacctcggcttctccggctcatgggaagcttggccgtatgaagcaggtgggctgagcctgcaccctgaagaccagagccctgagggccccacgcagtgacaaaggagagcccactatctcctgttttcagtttcacttttaccatcgttaaaagaagagcagttttggtgcatttttcaacctctcaacaaaaacacacacggaagaagattccaacagcaccctgctcttgctgggacctgctccgtgacaatgcagccggggacggtcagagaccgacccaaggcccatgttgctgggacctgctccgtgacaatgcagccgggacggtccgagacagacccaaggcccaggccagatgcctgcacaagacttgctccgtgacaatgcagccggggacggtcagagacagacccaaggcctatgttgctgggacccgctccgtgacaatgcagctgggacggtcagagacagacccaaggcccaggccagacgcctgcacgagacctgctcttgctgggacctgctccgtgacaatgcagccggggacggtcagagacagacccaaggcccatgttgctgggacccgctccgtgacaatgcagctgggatggtcagagacagaaccaaggcccaggccagacgcctgcacgagacctgctcttgctgggacccactccgcgacaatgcagctgggatggtcagagacagacccaaggcccaggccagatgcctgcacaagacttgctctgtgacaatgccgctggggacagtcagagacagacccaaggcccatcttgctgggacctgctccatgacaatgcagctgggacggtcagagacagacccaaggcccatcgtgctgggactcgctccgtgacaatgcagctgggatggtcagagacagaaccaaggcccaggccagacgcctgcacgagacctgctcttgctgggacccactccgcgacaatgcagctgggatggtcagagacagacccaaggcccaggccagatgcctgcacaagacttgctctgtgacaatgccgctggggacagtcagagacagacccaaagcccatcttgctgggacctgctccatgacaatgcagctgggacggtcagagacagacccaaggcccatcgtgctgggacccgctccgcgacaatgcagctgggatggtcagagacagacccaaggcccaggccagatgcctgcacaagacttgctctgtgacaatgccgctggggacagtcagagacagacccaaagcccatcttgctgggacctgctccatgacaatgcagctgggacggtcagagacagacccaaggcccatcgtgctgggactcgctccgtgacaatgcagctgggatggtcagagacagaaccaaggcccaggccagacgcctgcacgagacctgctcttgctgggacccagctccatgacaatgcagctgggatggtcagagacagacccaaggcccaggacagacgcctgcacaagatcccacgcacagatgccccaccccacgagcaggacttctcagttggccgcaggggcactcagcgtggtgaccagcaagagacaaacagcagcactgctcaagaatccactgggcattgtggggaaaaaacagaggaaggggaagtaaggggagaaggaaatcaggtagaaaacccagaaatacagaagatgctagcgagtgagtgagcacgcactgtccatgccacatcctcagacagtgccgagccaagttcctccataccccatggcacagacacagcacaacgcgcctgggcatggccgtcacacccaaaccaccagtcactatgggacggctccgcacatgctcaggacagcctcagaatgctgtccactgtgtcgtcagctgcagcaggctcccagtcggtgccgggctctcctctgcgtccttcgtgactgtccagagggaaggctgaggtgccacgacatcccgccagctccaggcgtgcaccgggcgccagcaccattcccactgccgggctctgacttacagagggggtgggctggggtgggggagagctcctccagggctgctgtttgtgattttgtctagaggatgtttgagctgatgattccaatgtgatccgcaagaattaagtgaaaggcaagatgcagtgatctttgtgcattccaaaacggccgcttagcagaactccagtccaagttgaggtaagagaaaatgattagggtccaaagagtgaactacccagcacattagtggttaaagtgagaacctgcgtccaggcgctttcctggggactcctcctccacctcggagtctccgcatgtgctccgcgaccttttccttggctgcagaagagtctccaacctcggaaggactacagacaaaaaggttttggtccctagctgaggagaagttggctgggtttcagtgttcttggcagactttggggggcttacacttttcgatttgcagaagagaacagaagtgcgtctgtttacatcgcttgctggctccgccaccgcggaggccgccgccgccggcacatcgccactactggcgcgggtgggctctggagggcgtccgcttaccagtgcgctctgagtgcaagcgctatgtgattcattatcaaatgtgactcttttgaaaagtttactctgctctgggttgagttctactggtttgagggttggtggttctgaattagtctccgagtttgaaggaagaggtaatgcatctgatggttcaagtttagggggagatttatctccttcctcgcccgcctccggccccagcgcagctccgtcctcttcgaagccttccaagcctggccccgtgggcaggggctggctgtgctgctggctcagcttgtttcggagaagggcaatttcctttttgagcagctttgcccgcttgctccgggagccgctggacttcatagcgcaggtgaggtcgagcatgtccagcagctctctcagctgctcctccaggcccaggtgggctctgttggcggggtccagcaacctgtccacgtcttcccaggagaaaggccgccgcggtgccgcagcaggccgctcaggcaggtgcatccccgaggcctcttccaagccgatgctgtccacctcgcgccgggcctgcctcagaacaacacctccctgatcgcgcagcctcaccgcggctctatagaacacggtgtccctggcattgtacttcatgcagttatctataatgagatcaaaatcctcctcaaactcatggaggtttttatacccttgagcttctaaccgtttcctcattgtggcaaagtccatgggatgtttaatgtgatccaaataatctggtacctccttcagactcacgggctgcgcaaatatcctggcggggtccttgtcttgcagctggtccagcactgagcgcagcagcaccgtcagcggggtcagccgcagctccatggcgacctgctccaccttcacctgctcacgcttgagcttctcccgcttgcgcagcagctcgatcagcaggcgagcgcgctccaggtcgtgccgcagccgctgccagtacttcagcttctctttggcagccttcatctcctcatcattttctctctgctgtgagcttcgctgagactgcaggctggactgcagccgccgcagcaggggggccccgttcctggacagccgcttgagcagccagtagctgtgggctcgctccacaaactgcttcttccgctgaatggccacctgattcgcaatcctatttaacctctgcgggggaatataaggagcgcacacggtcggcaggaccgcgcagggctcagccagagctttcttagccttttttgccttcttcctgaccttggatgtggacctgaccgttttaaccgagctctcttttcgacagacgccatttttcatttcgacatccccgtaaatattcagaggcctccgggtgcagcctggaggcgtgtggacatcacagtaagcggtctttctgacggagaaggtggtgccaccgccagtcagttccttcacgggctccattttcatgtacaggccagccttctgggcacacgtcacatggaatgctgtgtagcagtttgctttgtggcactggatgcaggcacccacgcccttctgcttacagaggtagcatgtcagtttccaccgggctggagggatgttcctcaccccatcgatgggctcgatgaacaccgtgttggcaaagccgacctctgggatccacagggcacacaccacgtgaccccagcggtcgtcatctgtctttttgaaggcaccacccttgttggggcacagcacacagtcggcgggccgggcccgcgactgcaggcagtggcggcagagccactggccctcggggatgtagggcaccccgtagcactcctggtgcacggccaggttgcacatgtcgcagaagaggatcacgttgctgttctgacactccccgtccatgcagatgcagcacacggcgtcctcgtcgatcagagactgctgctcgccctgcttctggttctcgcagtgcgactccttctcgaagcggtccatcaggaactcaaacatgctctgcgacacggcggggacgcagtcgcccttgcgcttctcattgacgatctccagccaggcatagtcctcctcgtccatgtcatactccacctcgttgtccagttcctcggccgacttctcgatgaacttgtagtacacaggaggcctcctgggggcggacggagggctgtactccacgatgcgcaccttgggctccgggagggcactggccgaggccggcgtgccgtgggcgctggggagggcctcgtttttctttttgactctgttgtttttgtgacgcttagttcttaagcagacaggaggccgctcgctgttttccttgttgctgttgcactcactcatctcttgagcagtgaggtcatcttccaatatgatctccaggggatcaaaaatactgatcctgtgcaagcgcccttcaatttctatctctaccatcctttgagcttgagcgtaggtcagcgtttctcgcgtaggggagtgtttaacactgcatggggaagaaggatgcctcgctgcagagcctcgatgacatcgtcctttcctcctcatttggtaatgattac

SEQ ID NO: 16013 - RNA, 7776 nt, Homo sapiens
  source 1..7776: mol_type = other RNA
gctgggattacaggcatgagccatgacacccggccatgtgaatttttttatccaaaaagaaccccgttttcctgcctacctacctcatccttaaaaaatttttaaatctatttccaaaggaaattatgtaaatttgtaaatagagcatttctgtagaatttttttggaaacgatgtctcactctgtcaccaaggatggagtgcaatggactccatggctcactgcaaccttgacctcctgggctcaagtgatcctcctgcctcagcctcctgagtggctgggaggcatgttttgaagggaatggctggactgcgggattttccacccgcttcgtacgcttcccgtctgttctcaatgagcacgaccgacttttcaatacaggggctgaatcagcctccacccgcttcatacacttgctgtctgttctcaatgagcatgactgactgaaacagaggggctaaatcaagctcagaagggaatgcacagattgggcgggtgcactgctgccctccacagactcaagtcagacaccggctccgtctctcctggactggaatgtaccgtgacctccaagggaagctctgtgtttctcattttaacctcggtcattttaaggcaggaactgtggccagttgggggtgtcatactcatttctggcaagggaacaaataaatttaaaaacctacaggagaaggccttgagccacacgctgagctgccctggggctccacatgctccccatactcatcacagagtgggctcagaccctgcacactcaggccccgaagatgtctcaagagggaattaaaagtcccgtcctggcccccgagaacccctcaggagcagcgactccatccctactccaacctgagtgggtgaaggcaagggaagcccacccagctcgcatcagcagtggacggacggagcccagcacccctgccagcattcagcccacaggcccggagaggggtctgccaacgcgtgtgacccgtctccagagagcagccacgagcctggcgacccacaccccacagcccggcccccagcacactccagaccccaggtgcagggtgagcctgctccaggctgaacagacgcagcccagggcctgggtggggaggcttttagtagttactggttggccgagcaacggccacttgggggaagacgatgaccagtgcggccttcacaagactgcccagaggtgccagcctgagggccctagcacgagatcacccgcagctgtgccagcaccaacacagccaagccatgcacagaccactcagcagccacgacggccccggctccgtgtgcatggagtggggccaggaaggggattaaaacacaaggcaagtccttaattctcagaaagaggagaatgataaaatgcccctcttaattttcctaagcattcagtgagtgcgcgtatgacgcaagaacacacagaggttctgcgtgtcacccatgaaaatgtgacagcacccgggaagacgtgggcagcacagacaaacccagcccaaccgagacaccacccagcaggaggcctggcgggggtgggacagctgcaaggcttgctaacaggcggtctgggggctgcggcagtgcggggtcacccaggaagccaagaagccagaccaggacacagacacatcccgggaggctctgcagccaccgcctggagtccccagaacctcgggggagctgcaaggtggcctgcgctgcccggaccctcccagcctccacctggaccaccagaaaataatctaagacagctatggttctgagatctctcaatctcggccctgccaactcccgccctgggaggctcttccagccagctgggagatgtccaccatgacccgcacctcagcacccctgcaaggacctcagcccagaacattctgaagcccaggccagccttgaggtggggcccaacgtggggaacccagggcctaaggtctgcagagatgggtgcccggtccatgaggcatttgcaaacagcaggcactgaggccgagcccaagcctctaaatcatgtaaatagcaaggggcaactttcagcaactttttcagcacgaggtttttttttaacgctgaaagtaaagctggtgactgtgagaaatacgttaaaagaggcggcggctgccaggaaagagccgctgccccatcaacacaggagctgcacggaattcccacagcggccagggtccacccaccctcaagggccttcccagtgacctcctaggaggccaaagactgaacacagaaatgtccctctctgcccccaaaggagatggcgcaaaggtgtcccacagcccagccaagcgcagtccccggaagcctgcccgtcaccaggtacgtccacagcacacctgaaactgtcccgggaggtccccaaagggtcttctgagagactgaaggccacagcggctgagacaccgcccctccccacagggaagagaagccccagggcccacctggggaggcggaggcctgcaggtctgactgatgggccgtagtctcctctggtctcaggctcccagcccccaacccatgtggacaccacaaatcctccaggccacaggtgtaagaacaccaggccctgatcagtggctgccgagacacctgagggcacggagccatgggaacgcaaccccacaacacgggatacaagcccgcccctgcccgcccctgccgctggcacccaagctgccacctcggcttctccggctcatgggaagcttggccgtatgaagcaggtgggctgagcctgcaccctgaagaccagagccctgagggccccacgcagtgacaaaggagagcccactatctcctgttttcagtttcacttttaccatcgttaaaagaagagcagttttggtgcatttttcaacctctcaacaaaaacacacacggaagaagattccaacagcaccctgctcttgctgggacctgctccgtgacaatgcagccggggacggtcagagaccgacccaaggcccatgttgctgggacctgctccgtgacaatgcagccgggacggtccgagacagacccaaggcccaggccagatgcctgcacaagacttgctccgtgacaatgcagccggggacggtcagagacagacccaaggcctatgttgctgggacccgctccgtgacaatgcagctgggacggtcagagacagacccaaggcccaggccagacgcctgcacgagacctgctcttgctgggacctgctccgtgacaatgcagccggggacggtcagagacagacccaaggcccatgttgctgggacccgctccgtgacaatgcagctgggatggtcagagacagaaccaaggcccaggccagacgcctgcacgagacctgctcttgctgggacctgctccgtgacaatgcagccggggatggtcagaaacagacccaaggcccatcttgctgggacccactccgcgacaatgcagctgggatggtcagagacagacccaaggcccaggccagatgcctgcacaagacttgctctgtgacaatgccgctggggacagtcagagacagacccaaggcccatcttgctgggacccactccgcgacaatgcagctgggatggtcagagacagacccaaggcccaggccagatgcctgcacaagacttgctctgtgacaatgccgctggggacagtcagagacagacccaaagcccatcttgctgggacctgctccatgacaatgcagctgggacggtcagagacagacccaaggcccatcgtgctgggacccgctccgcgacaatgcagctgggatggtcagagacagacccaaggcccaggccagatgcctgcacaagacttgctctgtgacaatgccgctggggacagtcagagacagacccaaagcccatcttgctgggacctgctccatgacaatgcagctgggacggtcagagacagacccaaggcccatcgtgctgggactcgctccgtgacaatgcagctgggatggtcagagacagaaccaaggcccaggccagacgcctgcacgagacctgctcttgctgggacccagctccatgacaatgcagctgggatggtcagagacagacccaaggcccaggacagacgcctgcacaagatcccacgcacagatgccccaccccacgagcaggacttctcagttggccgcaggggcactcagcgtggtgaccagcaagagacaaacagcagcactgctcaagaatccactgggcattgtggggaaaaaacagaggaaggggaagtaaggggagaaggaaatcaggtagaaaacccagaaatacagaagatgctagcgagtgagtgagcacgcactgtccatgccacatcctcagacagtgccgagccaagttcctccataccccatggcacagacacagcacaacgcgcctgggcatggccgtcacacccaaaccaccagtcactatgggacggctccgcacatgctcaggacagcctcagaatgctgtccactgtgtcgtcagctgcagcaggctcccagtcggtgccgggctctcctctgcgtccttcgtgactgtccagagggaaggctgaggtgccacgacatcccgccagctccaggcgtgcaccgggcgccagcaccattcccactgccgggctctgacttacagagggggtgggctggggtgggggagagctcctccagggctgctgtttgtgattttgtctagaggatgtttgagctgatgattccaatgtgatccgcaagaattaagtgaaaggcaagatgcagtgatctttgtgcattccaaaacggccgcttagcagaactccagtccaagttgaggtaagagaaaatgattagggtccaaagagtgaactacccagcacattagtggttaaagtgagaacctgcgtccaggcgctttcctggggactcctcctccacctcggagtctccgcatgtgctccgcgaccttttccttggctgcagaagagtctccaacctcggaaggactacagacaaaaaggttttggtccctagctgaggagaagttggctgggtttcagtgttcttggcagactttggggggcttacacttttcgatttgcagaagagaacagaagtgcgtctgtttacatcgcttgctggctccgccaccgcggaggccgccgccgccggcacatcgccactactggcgcgggtgggctctggagggcgtccgcttaccagtgcgctctgagtgcaagcgctatgtgattcattatcaaatgtgactcttttgaaaagtttactctgctctgggttgagttctactggtttgagggttggtggttctgaattagtctccgagtttgaaggaagaggtaatgcatctgatggttcaagtttagggggagatttatctccttcctcgcccgcctccggccccagcgcagctccgtcctcttcgaagccttccaagcctggccccgtgggcaggggctggctgtgctgctggctcagcttgtttcggagaagggcaatttcctttttgagcagctttgcccgcttgctccgggagccgctggacttcatagcgcaggtgaggtcgagcatgtccagcagctctctcagctgctcctccaggcccaggtgggctctgttggcggggtccagcaacctgtccacgtcttcccaggagaaaggccgccgcggtgccgcagcaggccgctcaggcaggtgcatccccgaggcctcttccaagccgatgctgtccacctcgcgccgggcctgcctcagaacaacacctccctgatcgcgcagcctcaccgcggctctatagaacacggtgtccctggcattgtacttcatgcagttatctataatgagatcaaaatcctcctcaaactcatggaggtttttatacccttgagcttctaaccgtttcctcattgtggcaaagtccatgggatgtttaatgtgatccaaataatctggtacctccttcagactcacgggctgcgcaaatatcctggcggggtccttgtcttgcagctggtccagcactgagcgcagcagcaccgtcagcggggtcagccgcagctccatggcgacctgctccaccttcacctgctcacgcttgagcttctcccgcttgcgcagcagctcgatcagcaggcgagcgcgctccaggtcgtgccgcagccgctgccagtacttcagcttctctttggcagccttcatctcctcatcattttctctctgctgtgagcttcgctgagactgcaggctggactgcagccgccgcagcaggggggccccgttcctggacagccgcttgagcagccagtagctgtgggctcgctccacaaactgcttcttccgctgaatggccacctgattcgcaatcctatttaacctctgcgggggaatataaggagcgcacacggtcggcaggaccgcgcagggctcagccagagctttcttagccttttttgccttcttcctgaccttggatgtggacctgaccgttttaaccgagctctcttttcgacagacgccatttttcatttcgacatccccgtaaatattcagaggcctccgggtgcagcctggaggcgtgtggacatcacagtaagcggtctttctgacggagaaggtggtgccaccgccagtcagttccttcacgggctccattttcatgtacaggccagccttctgggcacacgtcacatggaatgctgtgtagcagtttgctttgtggcactggatgcaggcacccacgcccttctgcttacagaggtagcatgtcagtttccaccgggctggagggatgttcctcaccccatcgatgggctcgatgaacaccgtgttggcaaagccgacctctgggatccacagggcacacaccacgtgaccccagcggtcgtcatctgtctttttgaaggcaccacccttgttggggcacagcacacagtcggcgggccgggcccgcgactgcaggcagtggcggcagagccactggccctcggggatgtagggcaccccgtagcactcctggtgcacggccaggttgcacatgtcgcagaagaggatcacgttgctgttctgacactccccgtccatgcagatgcagcacacggcgtcctcgtcgatcagagactgctgctcgccctgcttctggttctcgcagtgcgactccttctcgaagcggtccatcaggaactcaaacatgctctgcgacacggcggggacgcagtcgcccttgcgcttctcattgacgatctccagccaggcatagtcctcctcgtccatgtcatactccacctcgttgtccagttcctcggccgacttctcgatgaacttgtagtacacaggaggcctcctgggggcggacggagggctgtactccacgatgcgcaccttgggctccgggagggcactggccgaggccggcgtgccgtgggcgctggggagggcctcgtttttctttttgactctgttgtttttgtgacgcttagttcttaagcagacaggaggccgctcgctgttttccttgttgctgttgcactcactcatctcttgagcagtgaggtcatcttccaatatgatctccaggggatcaaaaatactgatcctgtgcaagcgcccttcaatttctatctctaccatcctttgagcttgagcgtaggtcagcgtttctcgcgtaggggagtgtttaacactgcatggggaagaaggatgcctcgctgcagagcctcgatgacatcgtcctttcctcctcatttggtaatgattac

SEQ ID NO: 16014 - RNA, 7843 nt, Homo sapiens
  source 1..7843: mol_type = other RNA
gctgggattacaggcatgagccatgacacccggccatgtgaatttttttatccaaaaagaaccccgttttcctgcctacctacctcatccttaaaaaatttttaaatctatttccaaaggaaattatgtaaatttgtaaatagagcatttctgtagaatttttttggaaacgatgtctcactctgtcaccaaggatggagtgcaatggactccatggctcactgcaaccttgacctcctgggctcaagtgatcctcctgcctcagcctcctgagtggctgggaggcatgttttgaagggaatggctggactgcgggattttccacccgcttcgtacgcttcccgtctgttctcaatgagcacgaccgacttttcaatacaggggctgaatcagcctccacccgcttcatacacttgctgtctgttctcaatgagcatgactgactgaaacagaggggctaaatcaagctcagaagggaatgcacagattgggcgggtgcactgctgccctccacagactcaagtcagacaccggctccgtctctcctggactggaatgtaccgtgacctccaagggaagctctgtgtttctcattttaacctcggtcattttaaggcaggaactgtggccagttgggggtgtcatactcatttctggcaagggaacaaataaatttaaaaacctacaggagaaggccttgagccacacgctgagctgccctggggctccacatgctccccatactcatcacagagtgggctcagaccctgcacactcaggccccgaagatgtctcaagagggaattaaaagtcccgtcctggcccccgagaacccctcaggagcagcgactccatccctactccaacctgagtgggtgaaggcaagggaagcccacccagctcgcatcagcagtggacggacggagcccagcacccctgccagcattcagcccacaggcccggagaggggtctgccaacgcgtgtgacccgtctccagagagcagccacgagcctggcgacccacaccccacagcccggcccccagcacactccagaccccaggtgcagggtgagcctgctccaggctgaacagacgcagcccagggcctgggtggggaggcttttagtagttactggttggccgagcaacggccacttgggggaagacgatgaccagtgcggccttcacaagactgcccagaggtgccagcctgagggccctagcacgagatcacccgcagctgtgccagcaccaacacagccaagccatgcacagaccactcagcagccacgacggccccggctccgtgtgcatggagtggggccaggaaggggattaaaacacaaggcaagtccttaattctcagaaagaggagaatgataaaatgcccctcttaattttcctaagcattcagtgagtgcgcgtatgacgcaagaacacacagaggttctgcgtgtcacccatgaaaatgtgacagcacccgggaagacgtgggcagcacagacaaacccagcccaaccgagacaccacccagcaggaggcctggcgggggtgggacagctgcaaggcttgctaacaggcggtctgggggctgcggcagtgcggggtcacccaggaagccaagaagccagaccaggacacagacacatcccgggaggctctgcagccaccgcctggagtccccagaacctcgggggagctgcaaggtggcctgcgctgcccggaccctcccagcctccacctggaccaccagaaaataatctaagacagctatggttctgagatctctcaatctcggccctgccaactcccgccctgggaggctcttccagccagctgggagatgtccaccatgacccgcacctcagcacccctgcaaggacctcagcccagaacattctgaagcccaggccagccttgaggtggggcccaacgtggggaacccagggcctaaggtctgcagagatgggtgcccggtccatgaggcatttgcaaacagcaggcactgaggccgagcccaagcctctaaatcatgtaaatagcaaggggcaactttcagcaactttttcagcacgaggtttttttttaacgctgaaagtaaagctggtgactgtgagaaatacgttaaaagaggcggcggctgccaggaaagagccgctgccccatcaacacaggagctgcacggaattcccacagcggccagggtccacccaccctcaagggccttcccagtgacctcctaggaggccaaagactgaacacagaaatgtccctctctgcccccaaaggagatggcgcaaaggtgtcccacagcccagccaagcgcagtccccggaagcctgcccgtcaccaggtacgtccacagcacacctgaaactgtcccgggaggtccccaaagggtcttctgagagactgaaggccacagcggctgagacaccgcccctccccacagggaagagaagccccagggcccacctggggaggcggaggcctgcaggtctgactgatgggccgtagtctcctctggtctcaggctcccagcccccaacccatgtggacaccacaaatcctccaggccacaggtgtaagaacaccaggccctgatcagtggctgccgagacacctgagggcacggagccatgggaacgcaaccccacaacacgggatacaagcccgcccctgcccgcccctgccgctggcacccaagctgccacctcggcttctccggctcatgggaagcttggccgtatgaagcaggtgggctgagcctgcaccctgaagaccagagccctgagggccccacgcagtgacaaaggagagcccactatctcctgttttcagtttcacttttaccatcgttaaaagaagagcagttttggtgcatttttcaacctctcaacaaaaacacacacggaagaagattccaacagcaccctgctcttgctgggacctgctccgtgacaatgcagccggggacggtcagagaccgacccaaggcccatgttgctgggacctgctccgtgacaatgcagccgggacggtccgagacagacccaaggcccaggccagatgcctgcacaagacttgctccgtgacaatgcagccggggacggtcagagacagacccaaggcctatgttgctgggacccgctccgtgacaatgcagctgggacggtcagagacagacccaaggcccaggccagacgcctgcacgagacctgctcttgctgggacctgctccgtgacaatgcagccggggacggtcagagacagacccaaggcccatgttgctgggacccgctccgtgacaatgcagctgggatggtcagagacagaaccaaggcccaggccagacgcctgcacgagacctgctcttgctgggacctgctccgtgacaatgcagccggggatggtcagaaacagacccaaggcccatcttgctgggacccactccgcgacaatgcagctgggatggtcagagacagacccaaggcccaggccagatgcctgcacaagacttgctctgtgacaatgccgctggggacagtcagagacagacccaaggcccatcttgctgggacctgctccatgacaatgcagctgggacggtcagagacagacccaaggcccatcgtgctgggactcgctccgtgacaatgcagctgggatggtcagagacagaaccaaggcccaggccagacgcctgcacgagacctgctcttgctgggacccactccgcgacaatgcagctgggatggtcagagacagacccaaggcccaggccagatgcctgcacaagacttgctctgtgacaatgccgctggggacagtcagagacagacccaaagcccatcttgctgggacctgctccatgacaatgcagctgggacggtcagagacagacccaaggcccatcgtgctgggacccgctccgcgacaatgcagctgggatggtcagagacagacccaaggcccaggccagatgcctgcacaagacttgctctgtgacaatgccgctggggacagtcagagacagacccaaagcccatcttgctgggacctgctccatgacaatgcagctgggacggtcagagacagacccaaggcccatcgtgctgggactcgctccgtgacaatgcagctgggatggtcagagacagaaccaaggcccaggccagacgcctgcacgagacctgctcttgctgggacccagctccatgacaatgcagctgggatggtcagagacagacccaaggcccaggacagacgcctgcacaagatcccacgcacagatgccccaccccacgagcaggacttctcagttggccgcaggggcactcagcgtggtgaccagcaagagacaaacagcagcactgctcaagaatccactgggcattgtggggaaaaaacagaggaaggggaagtaaggggagaaggaaatcaggtagaaaacccagaaatacagaagatgctagcgagtgagtgagcacgcactgtccatgccacatcctcagacagtgccgagccaagttcctccataccccatggcacagacacagcacaacgcgcctgggcatggccgtcacacccaaaccaccagtcactatgggacggctccgcacatgctcaggacagcctcagaatgctgtccactgtgtcgtcagctgcagcaggctcccagtcggtgccgggctctcctctgcgtccttcgtgactgtccagagggaaggctgaggtgccacgacatcccgccagctccaggcgtgcaccgggcgccagcaccattcccactgccgggctctgacttacagagggggtgggctggggtgggggagagctcctccagggctgctgtttgtgattttgtctagaggatgtttgagctgatgattccaatgtgatccgcaagaattaagtgaaaggcaagatgcagtgatctttgtgcattccaaaacggccgcttagcagaactccagtccaagttgaggtaagagaaaatgattagggtccaaagagtgaactacccagcacattagtggttaaagtgagaacctgcgtccaggcgctttcctggggactcctcctccacctcggagtctccgcatgtgctccgcgaccttttccttggctgcagaagagtctccaacctcggaaggaacttttcgatttgcagaagagaacagaagtgcgtctgtttacatcgcttgctggctccgccaccgcggaggccgccgccgccggcacatcgccactactggcgcgggtgggctctggagggcgtccgcttaccagtgcgctctgagtgcaagcgctatgtgattcattatcaaatgtgactcttttgaaaagtttactctgctctgggttgagttctactggtttgagggttggtggttctgaattagtctccgagtttgaaggaagaggtaatgcatctgatggttcaagtttagggggagatttatctccttcctcgcccgcctccggccccagcgcagctccgtcctcttcgaagccttccaagcctggccccgtgggcaggggctggctgtgctgctggctcagcttgtttcggagaagggcaatttcctttttgagcagctttgcccgcttgctccgggagccgctggacttcatagcgcaggtgaggtcgagcatgtccagcagctctctcagctgctcctccaggcccaggtgggctctgttggcggggtccagcaacctgtccacgtcttcccaggagaaaggccgccgcggtgccgcagcaggccgctcaggcaggtgcatccccgaggcctcttccaagccgatgctgtccacctcgcgccgggcctgcctcagaacaacacctccctgatcgcgcagcctcaccgcggctctatagaacacggtgtccctggcattgtacttcatgcagttatctataatgagatcaaaatcctcctcaaactcatggaggtttttatacccttgagcttctaaccgtttcctcattgtggcaaagtccatgggatgtttaatgtgatccaaataatctggtacctccttcagactcacgggctgcgcaaatatcctggcggggtccttgtcttgcagctggtccagcactgagcgcagcagcaccgtcagcggggtcagccgcagctccatggcgacctgctccaccttcacctgctcacgcttgagcttctcccgcttgcgcagcagctcgatcagcaggcgagcgcgctccaggtcgtgccgcagccgctgccagtacttcagcttctctttggcagccttcatctcctcatcattttctctctgctgtgagcttcgctgagactgcaggctggactgcagccgccgcagcaggggggccccgttcctggacagccgcttgagcagccagtagctgtgggctcgctccacaaactgcttcttccgctgaatggccacctgattcgcaatcctatttaacctctgcgggggaatataaggagcgcacacggtcggcaggaccgcgcagggctcagccagagctttcttagccttttttgccttcttcctgaccttggatgtggacctgaccgttttaaccgagctctcttttcgacagacgccatttttcatttcgacatccccgtaaatattcagaggcctccgggtgcagcctggaggcgtgtggacatcacagtaagcggtctttctgacggagaaggtggtgccaccgccagtcagttccttcacgggctccattttcatgtacaggccagccttctgggcacacgtcacatggaatgctgtgtagcagtttgctttgtggcactggatgcaggcacccacgcccttctgcttacagaggtagcatgtcagtttccaccgggctggagggatgttcctcaccccatcgatgggctcgatgaacaccgtgttggcaaagccgacctctgggatccacagggcacacaccacgtgaccccagcggtcgtcatctgtctttttgaaggcaccacccttgttggggcacagcacacagtcggcgggccgggcccgcgactgcaggcagtggcggcagagccactggccctcggggatgtagggcaccccgtagcactcctggtgcacggccaggttgcacatgtcgcagaagaggatcacgttgctgttctgacactccccgtccatgcagatgcagcacacggcgtcctcgtcgatcagagactgctgctcgccctgcttctggttctcgcagtgcgactccttctcgaagcggtccatcaggaactcaaacatgctctgcgacacggcggggacgcagtcgcccttgcgcttctcattgacgatctccagccaggcatagtcctcctcgtccatgtcatactccacctcgttgtccagttcctcggccgacttctcgatgaacttgtagtacacaggaggcctcctgggggcggacggagggctgtactccacgatgcgcaccttgggctccgggagggcactggccgaggccggcgtgccgtgggcgctggggagggcctcgtttttctttttgactctgttgtttttgtgacgcttagttcttaagcagacaggaggccgctcgctgttttccttgttgctgttgcactcactcatctcttgagcagtgaggtcatcttccaatatgatctccaggggatcaaaaatactgatcctgtgcaagcgcccttcaatttctatctctaccatcctttgagcttgagcgtaggtcagcgtttctcgcgtaggggagtgtttaacactgcatggggaagaaggatgcctcgctgcagagcctcgatgacatcgtcctttcctcctcatttggtaatgattac

SEQ ID NO: 16015 - RNA, 7925 nt, Homo sapiens
  source 1..7925: mol_type = other RNA
gctgggattacaggcatgagccatgacacccggccatgtgaatttttttatccaaaaagaaccccgttttcctgcctacctacctcatccttaaaaaatttttaaatctatttccaaaggaaattatgtaaatttgtaaatagagcatttctgtagaatttttttggaaacgatgtctcactctgtcaccaaggatggagtgcaatggactccatggctcactgcaaccttgacctcctgggctcaagtgatcctcctgcctcagcctcctgagtggctgggaggcatgttttgaagggaatggctggactgcgggattttccacccgcttcgtacgcttcccgtctgttctcaatgagcacgaccgacttttcaatacaggggctgaatcagcctccacccgcttcatacacttgctgtctgttctcaatgagcatgactgactgaaacagaggggctaaatcaagctcagaagggaatgcacagattgggcgggtgcactgctgccctccacagactcaagtcagacaccggctccgtctctcctggactggaatgtaccgtgacctccaagggaagctctgtgtttctcattttaacctcggtcattttaaggcaggaactgtggccagttgggggtgtcatactcatttctggcaagggaacaaataaatttaaaaacctacaggagaaggccttgagccacacgctgagctgccctggggctccacatgctccccatactcatcacagagtgggctcagaccctgcacactcaggccccgaagatgtctcaagagggaattaaaagtcccgtcctggcccccgagaacccctcaggagcagcgactccatccctactccaacctgagtgggtgaaggcaagggaagcccacccagctcgcatcagcagtggacggacggagcccagcacccctgccagcattcagcccacaggcccggagaggggtctgccaacgcgtgtgacccgtctccagagagcagccacgagcctggcgacccacaccccacagcccggcccccagcacactccagaccccaggtgcagggtgagcctgctccaggctgaacagacgcagcccagggcctgggtggggaggcttttagtagttactggttggccgagcaacggccacttgggggaagacgatgaccagtgcggccttcacaagactgcccagaggtgccagcctgagggccctagcacgagatcacccgcagctgtgccagcaccaacacagccaagccatgcacagaccactcagcagccacgacggccccggctccgtgtgcatggagtggggccaggaaggggattaaaacacaaggcaagtccttaattctcagaaagaggagaatgataaaatgcccctcttaattttcctaagcattcagtgagtgcgcgtatgacgcaagaacacacagaggttctgcgtgtcacccatgaaaatgtgacagcacccgggaagacgtgggcagcacagacaaacccagcccaaccgagacaccacccagcaggaggcctggcgggggtgggacagctgcaaggcttgctaacaggcggtctgggggctgcggcagtgcggggtcacccaggaagccaagaagccagaccaggacacagacacatcccgggaggctctgcagccaccgcctggagtccccagaacctcgggggagctgcaaggtggcctgcgctgcccggaccctcccagcctccacctggaccaccagaaaataatctaagacagctatggttctgagatctctcaatctcggccctgccaactcccgccctgggaggctcttccagccagctgggagatgtccaccatgacccgcacctcagcacccctgcaaggacctcagcccagaacattctgaagcccaggccagccttgaggtggggcccaacgtggggaacccagggcctaaggtctgcagagatgggtgcccggtccatgaggcatttgcaaacagcaggcactgaggccgagcccaagcctctaaatcatgtaaatagcaaggggcaactttcagcaactttttcagcacgaggtttttttttaacgctgaaagtaaagctggtgactgtgagaaatacgttaaaagaggcggcggctgccaggaaagagccgctgccccatcaacacaggagctgcacggaattcccacagcggccagggtccacccaccctcaagggccttcccagtgacctcctaggaggccaaagactgaacacagaaatgtccctctctgcccccaaaggagatggcgcaaaggtgtcccacagcccagccaagcgcagtccccggaagcctgcccgtcaccaggtacgtccacagcacacctgaaactgtcccgggaggtccccaaagggtcttctgagagactgaaggccacagcggctgagacaccgcccctccccacagggaagagaagccccagggcccacctggggaggcggaggcctgcaggtctgactgatgggccgtagtctcctctggtctcaggctcccagcccccaacccatgtggacaccacaaatcctccaggccacaggtgtaagaacaccaggccctgatcagtggctgccgagacacctgagggcacggagccatgggaacgcaaccccacaacacgggatacaagcccgcccctgcccgcccctgccgctggcacccaagctgccacctcggcttctccggctcatgggaagcttggccgtatgaagcaggtgggctgagcctgcaccctgaagaccagagccctgagggccccacgcagtgacaaaggagagcccactatctcctgttttcagtttcacttttaccatcgttaaaagaagagcagttttggtgcatttttcaacctctcaacaaaaacacacacggaagaagattccaacagcaccctgctcttgctgggacctgctccgtgacaatgcagccggggacggtcagagaccgacccaaggcccatgttgctgggacctgctccgtgacaatgcagccgggacggtccgagacagacccaaggcccaggccagatgcctgcacaagacttgctccgtgacaatgcagccggggacggtcagagacagacccaaggcctatgttgctgggacccgctccgtgacaatgcagctgggacggtcagagacagacccaaggcccaggccagacgcctgcacgagacctgctcttgctgggacctgctccgtgacaatgcagccggggacggtcagagacagacccaaggcccatgttgctgggacccgctccgtgacaatgcagctgggatggtcagagacagaaccaaggcccaggccagacgcctgcacgagacctgctcttgctgggacctgctccgtgacaatgcagccggggatggtcagaaacagacccaaggcccatcttgctgggacccactccgcgacaatgcagctgggatggtcagagacagacccaaggcccaggccagatgcctgcacaagacttgctctgtgacaatgccgctggggacagtcagagacagacccaaggcccatcttgctgggacctgctccatgacaatgcagctgggacggtcagagacagacccaaggcccatcgtgctgggactcgctccgtgacaatgcagctgggatggtcagagacagaaccaaggcccaggccagacgcctgcacgagacctgctcttgctgggacccactccgcgacaatgcagctgggatggtcagagacagacccaaggcccaggccagatgcctgcacaagacttgctctgtgacaatgccgctggggacagtcagagacagacccaaagcccatcttgctgggacctgctccatgacaatgcagctgggacggtcagagacagacccaaggcccatcgtgctgggacccgctccgcgacaatgcagctgggatggtcagagacagacccaaggcccaggccagatgcctgcacaagacttgctctgtgacaatgccgctggggacagtcagagacagacccaaagcccatcttgctgggacctgctccatgacaatgcagctgggacggtcagagacagacccaaggcccatcgtgctgggactcgctccgtgacaatgcagctgggatggtcagagacagaaccaaggcccaggccagacgcctgcacgagacctgctcttgctgggacccagctccatgacaatgcagctgggatggtcagagacagacccaaggcccaggacagacgcctgcacaagatcccacgcacagatgccccaccccacgagcaggacttctcagttggccgcaggggcactcagcgtggtgaccagcaagagacaaacagcagcactgctcaagaatccactgggcattgtggggaaaaaacagaggaaggggaagtaaggggagaaggaaatcaggtagaaaacccagaaatacagaagatgctagcgagtgagtgagcacgcactgtccatgccacatcctcagacagtgccgagccaagttcctccataccccatggcacagacacagcacaacgcgcctgggcatggccgtcacacccaaaccaccagtcactatgggacggctccgcacatgctcaggacagcctcagaatgctgtccactgtgtcgtcagctgcagcaggctcccagtcggtgccgggctctcctctgcgtccttcgtgactgtccagagggaaggctgaggtgccacgacatcccgccagctccaggcgtgcaccgggcgccagcaccattcccactgccgggctctgacttacagagggggtgggctggggtgggggagagctcctccagggctgctgtttgtgattttgtctagaggatgtttgagctgatgattccaatgtgatccgcaagaattaagtgaaaggcaagatgcagtgatctttgtgcattccaaaacggccgcttagcagaactccagtccaagttgaggtaagagaaaatgattagggtccaaagagtgaactacccagcacattagtggttaaagtgagaacctgcgtccaggcgctttcctggggactcctcctccacctcggagtctccgcatgtgctccgcgaccttttccttggctgcagaagagtctccaacctcggaaggactacagacaaaaaggttttggtccctagctgaggagaagttggctgggtttcagtgttcttggcagactttggggggcttacacttttcgatttgcagaagagaacagaagtgcgtctgtttacatcgcttgctggctccgccaccgcggaggccgccgccgccggcacatcgccactactggcgcgggtgggctctggagggcgtccgcttaccagtgcgctctgagtgcaagcgctatgtgattcattatcaaatgtgactcttttgaaaagtttactctgctctgggttgagttctactggtttgagggttggtggttctgaattagtctccgagtttgaaggaagaggtaatgcatctgatggttcaagtttagggggagatttatctccttcctcgcccgcctccggccccagcgcagctccgtcctcttcgaagccttccaagcctggccccgtgggcaggggctggctgtgctgctggctcagcttgtttcggagaagggcaatttcctttttgagcagctttgcccgcttgctccgggagccgctggacttcatagcgcaggtgaggtcgagcatgtccagcagctctctcagctgctcctccaggcccaggtgggctctgttggcggggtccagcaacctgtccacgtcttcccaggagaaaggccgccgcggtgccgcagcaggccgctcaggcaggtgcatccccgaggcctcttccaagccgatgctgtccacctcgcgccgggcctgcctcagaacaacacctccctgatcgcgcagcctcaccgcggctctatagaacacggtgtccctggcattgtacttcatgcagttatctataatgagatcaaaatcctcctcaaactcatggaggtttttatacccttgagcttctaaccgtttcctcattgtggcaaagtccatgggatgtttaatgtgatccaaataatctggtacctccttcagactcacgggctgcgcaaatatcctggcggggtccttgtcttgcagctggtccagcactgagcgcagcagcaccgtcagcggggtcagccgcagctccatggcgacctgctccaccttcacctgctcacgcttgagcttctcccgcttgcgcagcagctcgatcagcaggcgagcgcgctccaggtcgtgccgcagccgctgccagtacttcagcttctctttggcagccttcatctcctcatcattttctctctgctgtgagcttcgctgagactgcaggctggactgcagccgccgcagcaggggggccccgttcctggacagccgcttgagcagccagtagctgtgggctcgctccacaaactgcttcttccgctgaatggccacctgattcgcaatcctatttaacctctgcgggggaatataaggagcgcacacggtcggcaggaccgcgcagggctcagccagagctttcttagccttttttgccttcttcctgaccttggatgtggacctgaccgttttaaccgagctctcttttcgacagacgccatttttcatttcgacatccccgtaaatattcagaggcctccgggtgcagcctggaggcgtgtggacatcacagtaagcggtctttctgacggagaaggtggtgccaccgccagtcagttccttcacgggctccattttcatgtacaggccagccttctgggcacacgtcacatggaatgctgtgtagcagtttgctttgtggcactggatgcaggcacccacgcccttctgcttacagaggtagcatgtcagtttccaccgggctggagggatgttcctcaccccatcgatgggctcgatgaacaccgtgttggcaaagccgacctctgggatccacagggcacacaccacgtgaccccagcggtcgtcatctgtctttttgaaggcaccacccttgttggggcacagcacacagtcggcgggccgggcccgcgactgcaggcagtggcggcagagccactggccctcggggatgtagggcaccccgtagcactcctggtgcacggccaggttgcacatgtcgcagaagaggatcacgttgctgttctgacactccccgtccatgcagatgcagcacacggcgtcctcgtcgatcagagactgctgctcgccctgcttctggttctcgcagtgcgactccttctcgaagcggtccatcaggaactcaaacatgctctgcgacacggcggggacgcagtcgcccttgcgcttctcattgacgatctccagccaggcatagtcctcctcgtccatgtcatactccacctcgttgtccagttcctcggccgacttctcgatgaacttgtagtacacaggaggcctcctgggggcggacggagggctgtactccacgatgcgcaccttgggctccgggagggcactggccgaggccggcgtgccgtgggcgctggggagggcctcgtttttctttttgactctgttgtttttgtgacgcttagttcttaagcagacaggaggccgctcgctgttttccttgttgctgttgcactcactcatctcttgagcagtgaggtcatcttccaatatgatctccaggggatcaaaaatactgatcctgtgcaagcgcccttcaatttctatctctaccatcctttgagcttgagcgtaggtcagcgtttctcgcgtaggggagtgtttaacactgcatggggaagaaggatgcctcgctgcagagcctcgatgacatcgtcctttcctcctcatttggtaatgattac

SEQ ID NO: 16016 - RNA, 2581 nt, Homo sapiens
  source 1..2581: mol_type = other RNA
gctgggattacaggcatgagccatgcacccctacttctttagtgggagtctgtgccacagctgtggacacaggtgtccctagttattaaattagactttgtggtattttccccatcaggatgttcacacttccatgtggctaaagctattgatcttttctgttctggctcctgagctgagattttcttaaactctttctggatgaaatctttatttcatcaggctggtggcgtccacggcctcaactttacctccgtgatggaagagggggatctgaggctcccaggtgggccggcgccgccactcagggtgggccaggcgtccacaggctgggggcgggctggaggacagtggcagccccaggtggccacacagcatggtggtggtggtggtggtggtgcacggcaggcagccttggcctggcagctcgtgggaccctcgggggcacatgtggcgggtcctgcagggctgggggcagggccttgagcatccagttctgcaggaccaactggtgcacctgtgcgttctgcagcagcagcagctccaccatgtcttccttaatacttcctgaccgttgagtagggaaggcctggggaggaggaatctgtgctatgagtggctgctgagggagctgctgaatgatggtggcaggaggctgggggaccgtaggcaggatgatccttggcgggtctggggccagcggggatggggaggcagtgggtaggatgcccgtggggggcagctctgggggcagggctgacccgagggctcctctgcttggcccgctccaggcctgggcccgagagagctcgtccaggaggtgttgttcccggagtctctgcagaaggtccctccttctcttcagagcagtctgcagggcatcgtccggccggtcctcatttcctggctcgaggtggaggccctcaggtcccccttccacgttctgccgttcttgctccagcttctgtcccaagagcttcagcgtcagtcgggtcacttgctctgctgctgatgagtccagcatggtgggagctgcaggagacgactgtaggggcaggggaggccacagcccacctccctccctggttctgttactcgcaggaaagaactgctcagcaggagcccaagcaccggtgttgcctgcagggcgggccttacctcctggagaccagccacacagaagactgtggcctgagtcaggagaaggaagtttctggcggtcgagcttccacggcttcctgagggaggttgcagggagccgagatcgcgccattgcgctatagcctgggcgtcgcagcgagactgtctcaaaaaaagaaaaaaaattctgagcgagattccagggcttcctgagggcgcgtttaagttgcagttgctgaggaggctgcaaggtgagcttgcgtcagcgaggagccactccagcacgctcgggaagggcatcgttactgctgcaaacaagcacacggccctccacgacgaaccttttgcaagtgaaggcgcacgaacaggcccggaggactacaaagaaacccagaaaccagacttggacacatgaaataaaggggttagctgaaggaatactccacagttaaggacggcctgcgcgaggtcaccggccctgtcttggttttttgccacttcgctccagttagtttcccaagttccacctacgcgcgcgccagctgagaaaacgcccaccccggcggtcccgccacaggtcacaggcggtgcggaccccgggactgtgtccgggcttcggtgtccagagagctccaagacacccaaaccttccgtggtttccacctctgcaagcttatgttccgctgagctcaagctgagggacgacgacctcatgcgacgtcagtttccccctgggaccacgaacccacggccccatttctcttctgtctactaaaaaccttttcttttcttttttttttgagacctaagacatcagtgagacacacgagcagacacgggctcggtcgggaaaggcgggagctccaagcggcggggcctgcaggtccaggcggttcgcgggctttctgaccgcattcggccgagttcttctctgaagacccaggacccccggccgagggggcgcattcggcgggctggtggcgtaggattttgtttcgggttcccagggtcccggcaagggtgagggagcccttgcggatcccctgagatccacctcagcagcctcctccgtggtaggcctcaacttcccgcggcggcccacagccaacgactaatgcctgagcgggagaaaacggcctggccctgtccgggtggttgctgagcaccgttcggcgccgcccgcgcctgcagggagcccggcccgctgtcctggtggacacaaagcccaggggccgcccgcgcgggaccagcagcgcgaactttttgccgctcggccagcctggcaggggattttaaaatcggccaatcacagcgggcgccaggcctccgctttccgcttactggtcctgccgtaggaggcgggtacgtgagcgcaccaatctgtggccggcgagcgtaaagggcggggctccgcccaggctgcaccgcccagagcgcgcgt

SEQ ID NO: 16017 - RNA, 2654 nt, Homo sapiens
  source 1..2654: mol_type = other RNA
gctgggattacaggcatgagccatgcacccctacttctttagtgggagtctgtgccacagctgtggacacaggtgtccctagttattaaattagactttgtggtattttccccatcaggatgttcacacttccatgtggctaaagctattgatcttttctgttctggctcctgagctgagattttcttaaactctttctggatgaaatctttatttcatcaggctggtggcgtccacggcctcaactttacctccgtgatggaagagggggatctgaggctcccaggtgggccggcgccgccactcagggtgggccaggcgtccacaggctgggggcgggctggaggacagtggcagccccaggtggccacacagcatggtggtggtggtggtggtggtgcacggcaggcagccttggcctggcagctcgtgggaccctcgggggcacatgtggcgggtcctgcagggctgggggcagggccttgagcatccagttctgcaggaccaactggtgcacctgtgcgttctgcagcagcagcagctccaccatgtcttccttaatacttcctgaccgttgagtagggaaggcctggggaggaggaatctgtgctatgagtggctgctgagggagctgctgaatgatggtggcaggaggctgggggaccgtaggcaggatgatccttggcgggtctggggccagcggggatggggaggcagtgggtaggatgcccgtggggggcagctctgggggcagggctgacccgagggctcctctgcttggcccgctccaggcctgggcccgagagagctcgtccaggaggtgttgttcctgcaaggccgatgcagagctgctgcacacggggacggggagccccaacgccacagaggcacccccagcatcaggctcaggccagcctgggccaggtacaggcgcctctccgggcaggatggccatgactggaagacccttccagggttatgtgcatgagggtggcctcccggagtctctgcagaaggtccctccttctcttcagagcagtctgcagggcatcgtccggccggtcctcatttcctggctcgaggtggaggccctcaggtcccccttccacgttctgccgttcttgctccagcttctgtgaggaagagagaccgtgacagagacggtggctccacgcaaaggccctgtgtgctccaggaatgactaagaggctttctgtcccaagagcttcagcgtcagtcgggtcacttgctctgctgctgatgagtccagcatggtgggagctgcaggagacgactgtaggggcaggggaggccacagcccacctccctccctggttctgttactcgcaggaaagaactgctcagcaggagcccaagcaccggtgttgcctgcagggcgggccttacctcctggagaccagccacacagaagactgtggcctgagtcaggagaaggaagtttctggcggtcgagcttccacggcttcctgagggaggttgcagggagccgagatcgcgccattgcgctatagcctgggcgtcgcagcgagactgtctcaaaaaaagaaaaaaaattctgagcgagattccagggcttcctgagggcgcgtttaagttgcagttgctgaggaggctgcaaggtgagcttgcgtcagcgaggagccactccagcacgctcgggaagggcatcgttactgctgcaaacaagcacacggccctccacgacgaaccttttgcaagtgaaggcgcacgaacaggcccggaggactacaaagaaacccagaaaccagacttggacacatgaaataaaggggttagctgaaggaatactccacagttaaggacggcctgcgcgaggtcaccggccctgtcttggttttttgccacttcgctccagttagtttcccaagttccacctacgcgcgcgccagctgagaaaacgcccaccccggcggtcccgccacaggtcacaggcggtgcggaccccgggactgtgtccgggcttcggtgtccagagagctccaagacacccaaaccttccgtggtttccacctctgcaagcttatgttccgctgagctcaagctgagggacgacgacctcatgcgacgtcagtttccccctgggaccacgaacccacggccccatttctcttctgtctactaaaaaccttttcttttcttttttttttgagacctaagacatcagtgagacacacgagcagacacgggctcggtcgggaaaggcgggagctccaagcggcggggcctgcaggtccaggcggttcgcgggctttctgaccgcattcggccgagttcttctctgaagacccaggacccccggccgagggggcgcattcggcgggctggtggcgtaggattttgtttcgggttcccagggtcccggcaagggtgagggagcccttgcggatcccctgagatccacctcagcagcctcctccgtggtaggcctcaacttcccgcggcggcccacagccaacgactaatgcctgagcgggagaaaacggcctggccctgtccgggtggttgctgagcaccgttcggcgccgcccgcgcctgcagggagcccggcccgctgtcctggtggacacaaagcccaggggccgcccgcgcgggaccagcagcgcgaacttttt

SEQ ID NO: 16018 - RNA, 2688 nt, Homo sapiens
  source 1..2688: mol_type = other RNA
gctgggattacaggcatgagccatgcacccctacttctttagtgggagtctgtgccacagctgtggacacaggtgtccctagttattaaattagactttgtggtattttccccatcaggatgttcacacttccatgtggctaaagctattgatcttttctgttctggctcctgagctgagattttcttaaactctttctggatgaaatctttatttcatcaggctggtggcgtccacggcctcaactttacctccgtgatggaagagggggatctgaggctcccaggtgggccggcgccgccctacaggaaaggaggggtccctgggaggggctgttgccctggtggggttcacaggcccctcactgcaggggacccggagcaagggatgccccctggaatggccccgtgaccagaaagcgagcctgcccagcttccccaggaggagcctgcagtccacactcgcgtagccactccgggtggtggcagggtctctccctgctcccttccatagtcccgccacagcccacagccctgaggaagcctgggggtggagggtgccccggccagggtctctgtgactcacactcagggtgggccaggcgtccacaggctgggggcgggctggaggacagtggcagccccaggtggccacacagcatggtggtggtggtggtggtggtgcacggcaggcagccttggcctggcagctcgtgggaccctcgggggcacatgtggcgggtcctgcagggctgggggcagggccttgagcatccagttctgcaggaccaactggtgcacctgtgcgttctgcagcagcagcagctccaccatgtcttccttaatacttcctgaccgttgagtagggaaggcctggggaggaggaatctgtgctatgagtggctgctgagggagctgctgaatgatggtggcaggaggctgggggaccgtaggcaggatgatccttggcgggtctggggccagcggggatggggaggcagtgggtaggatgcccgtggggggcagctctgggggcagggctgacccgagggctcctctgcttggcccgctccaggcctgggcccgagagagctcgtccaggaggtgttgttcccggagtctctgcagaaggtccctccttctcttcagagcagtctgcagggcatcgtccggccggtcctcatttcctggctcgaggtggaggccctcaggtcccccttccacgttctgccgttcttgctccagcttctgtcccaagagcttcagcgtcagtcgggtcacttgctctgctgctgatgagtccagcatggtgggagctgcaggagacgactgtaggggcaggggaggccacagcccacctccctccctggttctgttactcgcaggaaagaactgctcagcaggagcccaagcaccggtgttgcctgcagggcgggccttacctcctggagaccagccacacagaagactgtggcctgagtcaggagaaggaagtttctggcggtcgagcttccacggcttcctgagggaggttgcagggagccgagatcgcgccattgcgctatagcctgggcgtcgcagcgagactgtctcaaaaaaagaaaaaaaattctgagcgagattccagggcttcctgagggcgcgtttaagttgcagttgctgaggaggctgcaaggtgagcttgcgtcagcgaggagccactccagcacgctcgggaagggcatcgttactgctgcaaacaagcacacggccctccacgacgaaccttttgcaagtgaaggcgcacgaacaggcccggaggactacaaagaaacccagaaaccagacttggacacatgaaataaaggggttagctgaaggaatactccacagttaaggacggcctgcgcgaggtcaccggccctgtcttggttttttgccacttcgctccagttagtttcccaagttccacctacgcgcgcgccagctgagaaaacgcccaccccggcggtcccgccacaggtcacaggcggtgcggaccccgggactgtgtccgggcttcggtgtccagagagctccaagacacccaaaccttccgtggtttccacctctgcaagcttatgttccgctgagctcaagctgagggacgacgacctcatgcgacgtcagtttccccctgggaccacgaacccacggccccatttctcttctgtctactaaaaaccttttcttttcttttttttttgagacctaagacatcagtgagacacacgagcagacacgggctcggtcgggaaaggcgggagctccaagcggcggggcctgcaggtccaggcggttcgcgggctttctgaccgcattcggccgagttcttctctgaagacccaggacccccggccgagggggcgcattcggcgggctggtggcgtaggattttgtttcgggttcccagggtcccggcaagggtgagggagcccttgcggatcccctgagatccacctcagcagcctcctccgtggtaggcctcaacttcccgcggcggcccacagccaacgactaatgcctgagcgggagaaaacggcctggccctgtccgggtggttgctgagcaccgttcggcgccgcccgcgcctgcagggagcccggcccgctgtcctggtggacacaaagcccaggggccgcccgcgcgggaccagcagcgcgaacttttt

SEQ ID NO: 16019 - RNA, 4866 nt, Homo sapiens
  source 1..4866: mol_type = other RNA
gctgggattacaggcatgagccatgcacccctacttctttagtgggagtctgtgccacagctgtggacacaggtgtccctagttattaaattagactttgtggtattttccccatcaggatgttcacacttccatgtggctaaagctattgatcttttctgttctggctcctgagctgagattttcttaaactctttctggatgaaatctttatttcatcaggctggtggcgtccacggcctcaactttacctccgtgatggaagagggggatctgaggctcccaggtgggccggcgccgccctacaggaaaggaggggtccctgggaggggctgttgccctggtggggttcacaggcccctcactgcaggggacccggagcaagggatgccccctggaatggccccgtgaccagaaagcgagcctgcccagcttccccaggaggagcctgcagtccacactcgcgtagccactccgggtggtggcagggtctctccctgctcccttccatagtcccgccacagcccacagccctgaggaagcctgggggtggagggtgccccggccagggtctctgtgactcacactcagggtgggccaggcgtccacaggctgggggcgggctggaggacagtggcagccccaggtggccacacagcatggtggtggtggtggtggtggtgcacggcaggcagccttggcctggcagctcgtgggaccctcgggggcacatgtggcgggtcctgcagggctgggggcagggccttgagcatccagttctgcaggaccaactggtgcacctgtgcgttctgcagcagcagcagctccaccatgtcttccttaatacttcctgaccgttgagtagggaaggcctggggaggaggaatctgtgctatgagtggctgctgagggagctgctgaatgatggtggcaggaggctgggggaccgtaggcaggatgatccttggcgggtctggggccagcggggatggggaggcagtgggtaggatgcccgtggggggcagctctgggggcagggctgacccgagggctcctctgcttggcccgctccaggcctgggcccgagagagctcgtccaggaggtgttgttcccggagtctctgcagaaggtccctccttctcttcagagcagtctgcagggcatcgtccggccggtcctcatttcctggctcgaggtggaggccctcaggtcccccttccacgttctgccgttcttgctccagcttctgtcccaagagcttcagcgtcagtcgggtcacttgctctgctgctgatgagtccagcatggtgggagctgcaggagacgactgtaggggcaggggaggccacagcccacctccctccctggttctgttactcgcaggaaagaactgctcagcaggagcccaagcaccggtgttgcctgcagggcgggccttacctcctggagaccagccagagtactctatggccatgaaaagagcagaacaccaccaggtcaaagtggccgttttacagacagtcttgctgtcacttgtgagaagccctccacatctgctgctgcaggctctgcccacatcagagatgcttccttgccagattctccttttcgttgaactggttaactttttttcctctcctctttctcttgatgtggaatgtttataacatttatgcagtggtcaagtatactattatgtatggtttgtaatactgactgacttaaggagagacttgagcctgtgtgcccacagctgtgactgccaagtgaatgggaagcactaagaattgcctcctcgggatctctagtagtatacataacatgctccagagggcatggatttgtcagactttttttttaaatagggtttttaagaacagttttagatttagagtaattgagaagatagtacatggagatcccacataccacatgtgtggcttcccctcttattaacatcttaccttagtgtgctacatatgttatatatatatatattttttttgagacagagtctcgctgcgacgcccaggctagagtgcaatggtgcaatcttggctcactgcaacctctgcttcccagtttcaagcgattcttctgcctcagcctctcgagtagctgggactacaggtacgtgccatcatgcccagctaatttttgagtgaaagccagtgcacctggcccatttgttatgattaatgaaccaatattgagacacaagtaactgaagtccacactttgacagtttccttaggtttgcctcatgtccctaatgtggtatccatcagaacaccccattacattgagttatgtgtctttaggctccttctcagactttcctcgtttttgatgaccttgacagtttcgaagagtactgggcagatattttgaagaatgtccctcaattaaaatgtgtctattatctcctggttagactgggactgcaggttacagaaaggaagcatctaggggtgaagtgccactgtcaccccatcacatcagggacacacactgtcacctcgactataactgtgaggctgacctgcgtcacttggctgaggtggagtctgccagttttctccacaataaagtggctctttccctccttttctttattgcactctttgggaggaagtggctatgtgtggtctacacttaaggagaggggagttacgtttccctccttgagggtgagtatctacaaaatttatctgggcagcttttttttttttttttttttgagttagggtctcagtctgtcacccaggttggagtgcagtggttgcctggccttgacagctttttaatagtttaaaatgaattgaggctgggcgaggttgctcatgcctgtaactccagcactttgagaggccaaggcaggtggatcacttgagcccaggagttcaagaccagcctgggcaacacagtgagaccctgtgtctactaaaaatacaaaaattagctgggcatggtggtgtgcctgtaattccagctgctcaggaggctgacatggagaatcacctgagcccggggaagttgaggctgcaatgagcggtggtctcaccactgcactctagcctgtgtgacagactgagaccctgcctataaaaaagaaaagaaaaaagaactgaaataagacccaagtccaacattagcagaacctctctaggatgtccacagaaacgactctggggttctgaggaacacagtctaggcaaacctgggcacatcccctcagtcccacagttgtaaatgtattgtaacacgtaacagttgtgagattcaggcgcggtctgggtctctgttcctggaaagtgtgatcctgtgggtgcagcccctgctcgcttggctgtgttgcctgcctggcccctgctctaatgagcccactgcccagagtttgctcaaaccacccaattccgagtctgggaaccaggagaccgctggacaccccgctcaccacacagaagactgtggcctgagtcaggagaaggaagtttctggcggtcgagcttccacggcttcctgagggaggttgcagggagccgagatcgcgccattgcgctatagcctgggcgtcgcagcgagactgtctcaaaaaaagaaaaaaaattctgagcgagattccagggcttcctgagggcgcgtttaagttgcagttgctgaggaggctgcaaggtgagcttgcgtcagcgaggagccactccagcacgctcgggaagggcatcgttactgctgcaaacaagcacacggccctccacgacgaaccttttgcaagtgaaggcgcacgaacaggcccggaggactacaaagaaacccagaaaccagacttggacacatgaaataaaggggttagctgaaggaatactccacagttaaggacggcctgcgcgaggtcaccggccctgtcttggttttttgccacttcgctccagttagtttcccaagttccacctacgcgcgcgccagctgagaaaacgcccaccccggcggtcccgccacaggtcacaggcggtgcggaccccgggactgtgtccgggcttcggtgtccagagagctccaagacacccaaaccttccgtggtttccacctctgcaagcttatgttccgctgagctcaagctgagggacgacgacctcatgcgacgtcagtttccccctgggaccacgaacccacggccccatttctcttctgtctactaaaaaccttttcttttcttttttttttgagacctaagacatcagtgagacacacgagcagacacgggctcggtcgggaaaggcgggagctccaagcggcggggcctgcaggtccaggcggttcgcgggctttctgaccgcattcggccgagttcttctctgaagacccaggacccccggccgagggggcgcattcggcgggctggtggcgtaggattttgtttcgggttcccagggtcccggcaagggtgagggagcccttgcggatcccctgagatccacctcagcagcctcctccgtggtaggcctcaacttcccgcggcggcccacagccaacgactaatgcctgagcgggagaaaacggcctggccctgtccgggtggttgctgagcaccgttcggcgccgcccgcgcctgcagggagcccggcccgctgtcctggtggacacaaagcccaggggccgcccgcgcgggaccagcagcgcgaactttttgccgctcggccagcctggcaggggattttaaaatcggccaatcacagcgggcgccaggcctccgctttccgcttactggtcctgccgtaggaggcgggtacgtgagcgcaccaatctgtggccggcgagcgtaaagggcggggctccgcccaggctgcaccgcccagagcgcgcgt

SEQ ID NO: 16020 - RNA, 1855 nt, Homo sapiens
  source 1..1855: mol_type = other RNA
gctgggattacaggcatgagccatgcacccctacttctttagtgggagtctgtgccacagctgtggacacaggtgtccctagttattaaattagactttgtggtattttccccatcaggatgttcacacttccatgtggctaaagctattgatcttttctgttctggctcctgagctgagattttcttaaactctttctggatgaaatctttatttcatcaggctggtggcgtccacggcctcaactttacctccgtgatggaagagggggatctgaggctcccaggtgggccggcgccgccctacaggaaaggaggggtccctgggaggggctgttgccctggtggggttcacaggcccctcactgcaggggacccggagcaagggatgccccctggaatggccccgtgaccagaaagcgagcctgcccagcttccccaggaggagcctgcagtccacactcgcgtagccactccgggtggtggcagggtctctccctgctcccttccatagtcccgccacagcccacagccctgaggaagcctgggggtggagggtgccccggccagggtctctgtgactcacactcagggtgggccaggcgtccacaggctgggggcgggctggaggacagtggcagccccaggtggccacacagcatggtggtggtggtggtggtggtgcacggcaggcagccttggcctggcagctcgtgggaccctcgggggcacatgtggcgggtcctgcagggctgggggcagggccttgagcatccagttctgcaggaccaactggtgcacctgtgcgttctgcagcagcagcagctccaccatgtcttccttaatacttcctgaccgttgagtagggaaggcctggggaggaggaatctgtgctatgagtggctgctgagggagctgctgaatgatggtggcaggaggctgggggaccgtaggcaggatgatccttggcgggtctggggccagcggggatggggaggcagtgggtaggatgcccgtggggggcagctctgggggcagggctgacccgagggctcctctgcttggcccgctccaggcctgggcccgagagagctcgtccaggaggtgttgttcccggagtctctgcagaaggtccctccttctcttcagagcagtctgcagggcatcgtccggccggtcctcatttcctggctcgaggtggaggccctcaggtcccccttccacgttctgccgttcttgctccagcttctgtcccaagagcttcagcgtcagtcgggtcacttgctctgctgctgatgagtccagcatggtgggagctgcaggagacgactgtaggggcaggggaggccacagcccacctccctccctggttctgttactcgcaggaaagaactgctcagcaggagcccaagcaccggtgttgcctgcagggcgggccttacctcctggagaccagccttggggctgggggcactgggcagggagtcaagtttgcaggaagcttcgcagagggtgacgcaaaacaggagcgtggtctgcacttggttgggcattaaactccacgttgatgagttagtcaatcccactagcaggcagactgacatgtgggggatgtcagcagcaggggcccagacctgtggacccgaggggcagaggtcagcaccctcctcggtgcagctaacccaggaacttgcctcagtggccaaaattgctctcttgccctcagttctgtaaatggcccatgtccatcagtatctatggttgtgtgcctgtcctgtcttccaacccacatccatgtagggaccctgaagctggaccagtgagtgattgggtgaaggctggctagcccgtaggag

SEQ ID NO: 16021 - RNA, 1581 nt, Homo sapiens
  source 1..1581: mol_type = other RNA
gctgggattacaggcatgagccatgcacccctacttctttagtgggagtctgtgccacagctgtggacacaggtgtccctagttattaaattagactttgtggtattttccccatcaggatgttcacacttccatgtggctaaagctattgatcttttctgttctggctcctgagctgagattttcttaaactctttctggatgaaatctttatttcatcaggctggtggcgtccacggcctcaactttacctccgtgatggaagagggggatctgaggctcccaggtgggccggcgccgccctacaggaaaggaggggtccctgggaggggctgttgccctggtggggttcacaggcccctcactgcaggggacccggagcaagggatgccccctggaatggccccgtgaccagaaagcgagcctgcccagcttccccaggaggagcctgcagtccacactcgcgtagccactccgggtggtggcagggtctctccctgctcccttccatagtcccgccacagcccacagccctgaggaagcctgggggtggagggtgccccggccagggtctctgtgactcacactcagggtgggccaggcgtccacaggctgggggcgggctggaggacagtggcagccccaggtggccacacagcatggtggtggtggtggtggtggtgcacggcaggcagccttggcctggcagctcgtgggaccctcgggggcacatgtggcgggtcctgcagggctgggggcagggccttgagcatccagttctgcaggaccaactggtgcacctgtgcgttctgcagcagcagcagctccaccatgtcttccttaatacttcctgaccgttgagtagggaaggcctggggaggaggaatctgtgctatgagtggctgctgagggagctgctgaatgatggtggcaggaggctgggggaccgtaggcaggatgatccttggcgggtctggggccagcggggatggggaggcagtgggtaggatgcccgtggggggcagctctgggggcagggctgacccgagggctcctctgcttggcccgctccaggcctgggcccgagagagctcgtccaggaggtgttgttcccggagtctctgcagaaggtccctccttctcttcagagcagtctgcagggcatcgtccggccggtcctcatttcctggctcgaggtggaggccctcaggtcccccttccacgttctgccgttcttgctccagcttctgtgaggaagagagaccgtgacagagacggtggctccacgcaaaggccctgtgtgctccaggaatgactaagaggctttctgctgggtgtgtccaggggtgagtccctctcatggcggcctgtgggccaggatgcagggctggcgaaaggtgggcagcaggtccctcaggcagcaggagagggaacaatgcaggcagggggtgcagaggtgcccccaggcaccgaggctccccagaccctgtgctcagtggcctgtcccaagagcttcagcgtcagtcgggtcacttgctctgctgctgatgagtccagcatggtgggagctgcaggagacga

SEQ ID NO: 16022 - RNA, 1869 nt, Homo sapiens
  source 1..1869: mol_type = other RNA
gctgggattacaggcatgagccatgcacccctacttctttagtgggagtctgtgccacagctgtggacacaggtgtccctagttattaaattagactttgtggtattttccccatcaggatgttcacacttccatgtggctaaagctattgatcttttctgttctggctcctgagctgagattttcttaaactctttctggatgaaatctttatttcatcaggctggtggcgtccacggcctcaactttacctccgtgatggaagagggggatctgaggctcccaggtgggccggcgccgccctacaggaaaggaggggtccctgggaggggctgttgccctggtggggttcacaggcccctcactgcaggggacccggagcaagggatgccccctggaatggccccgtgaccagaaagcgagcctgcccagcttccccaggaggagcctgcagtccacactcgcgtagccactccgggtggtggcagggtctctccctgctcccttccatagtcccgccacagcccacagccctgaggaagcctgggggtggagggtgccccggccagggtctctgtgactcacactcagggtgggccaggcgtccacaggctgggggcgggctggaggacagtggcagccccaggtggccacacagcatggtggtggtggtggtggtggtgcacggcaggcagccttggcctggcagctcgtgggaccctcgggggcacatgtggcgggtcctgcagggctgggggcagggccttgagcatccagttctgcaggaccaactggtgcacctgtgcgttctgcagcagcagcagctccaccatgtcttccttaatacttcctgaccgttgagtagggaaggcctggggaggaggaatctgtgctatgagtggctgctgagggagctgctgaatgatggtggcaggaggctgggggaccgtaggcaggatgatccttggcgggtctggggccagcggggatggggaggcagtgggtaggatgcccgtggggggcagctctgggggcagggctgacccgagggctcctctgcttggcccgctccaggcctgggcccgagagagctcgtccaggaggtgttgttcctgcaaggccgatgcagagctgctgcacacggggacggggagccccaacgccacagaggcacccccagcatcaggctcaggccagcctgggccaggtacaggcgcctctccgggcaggatggccatgactggaagacccttccagggttatgtgcatgagggtggcctcccggagtctctgcagaaggtccctccttctcttcagagcagtctgcagggcatcgtccggccggtcctcatttcagcttgccccacgttccaaagaacaagaaatgctcctctggcctcctcagcttctccctggacgtccccgggtaacagtgaggacagcagctcctccccaaccaatggacaagctcagggtctggaaccagagcaactgggtctgatctgggtgcgaccactgccagggtgagcaacctctctgcctccattttctcatctggctcgaggtggaggccctcaggtcccccttccacgttctgccgttcttgctccagcttctgctgggtgtgtccaggggtgagtccctctcatggcggcctgtgggccaggatgcagggctggcgaaaggtgggcagcaggtccctcaggcagcaggagagggaacaatgcaggcagggggtgcagaggtgcccccaggcaccgaggctccccagaccctgtgctcagtggcctgtcccaagagcttcagcgtcagtcgggtcacttgctctgctgctgatgagtccagcatggtgggagctgcaggagacga

SEQ ID NO: 16023 - RNA, 2070 nt, Homo sapiens
  source 1..2070: mol_type = other RNA
gctgggattacaggcatgagccatgcacccctacttctttagtgggagtctgtgccacagctgtggacacaggtgtccctagttattaaattagactttgtggtattttccccatcaggatgttcacacttccatgtggctaaagctattgatcttttctgttctggctcctgagctgagattttcttaaactctttctggatgaaatctttatttcatcaggctggtggcgtccacggcctcaactttacctccgtgatggaagagggggatctgaggctcccaggtgggccggcgccgccctacaggaaaggaggggtccctgggaggggctgttgccctggtggggttcacaggcccctcactgcaggggacccggagcaagggatgccccctggaatggccccgtgaccagaaagcgagcctgcccagcttccccaggaggagcctgcagtccacactcgcgtagccactccgggtggtggcagggtctctccctgctcccttccatagtcccgccacagcccacagccctgaggaagcctgggggtggagggtgccccggccagggtctctgtgactcacactcagggtgggccaggcgtccacaggctgggggcgggctggaggacagtggcagccccaggtggccacacagcatggtggtggtggtggtggtggtgcacggcaggcagccttggcctggcagctcgtgggaccctcgggggcacatgtggcgggtcctgcagggctgggggcagggccttgagcatccagttctgcaggaccaactggtgcacctgtgcgttctgcagcagcagcagctccaccatgtcttccttaatacttcctgaccgttgagtagggaaggcctggggaggaggaatctgtgctatgagtggctgctgagggagctgctgaatgatggtggcaggaggctgggggaccgtaggcaggatgatccttggcgggtctggggccagcggggatggggaggcagtgggtaggatgcccgtggggggcagctctgggggcagggctgacccgagggctcctctgcttggcccgctccaggcctgggcccgagagagctcgtccaggaggtgttgttcctgcaaggccgatgcagagctgctgcacacggggacggggagccccaacgccacagaggcacccccagcatcaggctcaggccagcctgggccaggtacaggcgcctctccgggcaggatggccatgactggaagacccttccagggttatgtgcatgagggtggcctcccggagtctctgcagaaggtccctccttctcttcagagcagtctgcagggcatcgtccggccggtcctcatttcagcttgccccacgttccaaagaacaagaaatgctcctctggcctcctcagcttctccctggacgtccccgggtaacagtgaggacagcagctcctccccaaccaatggacaagctcagggtctggaaccagagcaactgggtctgatctgggtgcgaccactgccagggtgagcaacctctctgcctccattttctcatctggctcgaggtggaggccctcaggtcccccttccacgttctgccgttcttgctccagcttctgtcccaagagcttcagcgtcagtcgggtcacttgctctgctgctgatgagtccagcatggtgggagctgcaggagacgactgtaggggcaggggaggccacagcccacctccctccctggttctgttactcgcaggaaagaactgctcagcaggagcccaagcaccggtgttgcctgcagggcgggccttacctcctggagaccagccttggggctgggggcactgggcagggagtcaagtttgcaggaagcttcgcagagggtgacgcaaaacaggagcgtggtctgcacttggttgggcattaaactccacgttgatgagttagtcaatcccactagcaggcagactgacatgtgggggatgtcagcagcaggggcccagaccacacagaagactgtggcctgagtcaggagaaggaagtttctggcggtcgagcttccacggcttcctga

SEQ ID NO: 16024 - RNA, 3033 nt, Homo sapiens
  source 1..3033: mol_type = other RNA
gctgggattacaggcatgagccatgcacccctacttctttagtgggagtctgtgccacagctgtggacacaggtgtccctagttattaaattagactttgtggtattttccccatcaggatgttcacacttccatgtggctaaagctattgatcttttctgttctggctcctgagctgagattttcttaaactctttctggatgaaatctttatttcatcaggctggtggcgtccacggcctcaactttacctccgtgatggaagagggggatctgaggctcccaggtgggccggcgccgccctacaggaaaggaggggtccctgggaggggctgttgccctggtggggttcacaggcccctcactgcaggggacccggagcaagggatgccccctggaatggccccgtgaccagaaagcgagcctgcccagcttccccaggaggagcctgcagtccacactcgcgtagccactccgggtggtggcagggtctctccctgctcccttccatagtcccgccacagcccacagccctgaggaagcctgggggtggagggtgccccggccagggtctctgtgactcacactcagggtgggccaggcgtccacaggctgggggcgggctggaggacagtggcagccccaggtggccacacagcatggtggtggtggtggtggtggtgcacggcaggcagccttggcctggcagctcgtgggaccctcgggggcacatgtggcgggtcctgcagggctgggggcagggccttgagcatccagttctgcaggaccaactggtgcacctgtgcgttctgcagcagcagcagctccaccatgtcttccttaatacttcctgaccgttgagtagggaaggcctggggaggaggaatctgtgctatgagtggctgctgagggagctgctgaatgatggtggcaggaggctgggggaccgtaggcaggatgatccttggcgggtctggggccagcggggatggggaggcagtgggtaggatgcccgtggggggcagctctgggggcagggctgacccgagggctcctctgcttggcccgctccaggcctgggcccgagagagctcgtccaggaggtgttgttcctgcaaggccgatgcagagctgctgcacacggggacggggagccccaacgccacagaggcacccccagcatcaggctcaggccagcctgggccaggtacaggcgcctctccgggcaggatggccatgactggaagacccttccagggttatgtgcatgagggtggcctcccggagtctctgcagaaggtccctccttctcttcagagcagtctgcagggcatcgtccggccggtcctcatttcctggctcgaggtggaggccctcaggtcccccttccacgttctgccgttcttgctccagcttctgtcccaagagcttcagcgtcagtcgggtcacttgctctgctgctgatgagtccagcatggtgggagctgcaggagacgactgtaggggcaggggaggccacagcccacctccctccctggttctgttactcgcaggaaagaactgctcagcaggagcccaagcaccggtgttgcctgcagggcgggccttacctcctggagaccagccacacagaagactgtggcctgagtcaggagaaggaagtttctggcggtcgagcttccacggcttcctgagggaggttgcagggagccgagatcgcgccattgcgctatagcctgggcgtcgcagcgagactgtctcaaaaaaagaaaaaaaattctgagcgagattccagggcttcctgagggcgcgtttaagttgcagttgctgaggaggctgcaaggtgagcttgcgtcagcgaggagccactccagcacgctcgggaagggcatcgttactgctgcaaacaagcacacggccctccacgacgaaccttttgcaagtgaaggcgcacgaacaggcccggaggactacaaagaaacccagaaaccagacttggacacatgaaataaaggggttagctgaaggaatactccacagttaaggacggcctgcgcgaggtcaccggccctgtcttggttttttgccacttcgctccagttagtttcccaagttccacctacgcgcgcgccagctgagaaaacgcccaccccggcggtcccgccacaggtcacaggcggtgcggaccccgggactgtgtccgggcttcggtgtccagagagctccaagacacccaaaccttccgtggtttccacctctgcaagcttatgttccgctgagctcaagctgagggacgacgacctcatgcgacgtcagtttccccctgggaccacgaacccacggccccatttctcttctgtctactaaaaaccttttcttttcttttttttttgagacctaagacatcagtgagacacacgagcagacacgggctcggtcgggaaaggcgggagctccaagcggcggggcctgcaggtccaggcggttcgcgggctttctgaccgcattcggccgagttcttctctgaagacccaggacccccggccgagggggcgcattcggcgggctggtggcgtaggattttgtttcgggttcccagggtcccggcaagggtgagggagcccttgcggatcccctgagatccacctcagcagcctcctccgtggtaggcctcaacttcccgcggcggcccacagccaacgactaatgcctgagcgggagaaaacggcctggccctgtccgggtggttgctgagcaccgttcggcgccgcccgcgcctgcagggagcccggcccgctgtcctggtggacacaaagcccaggggccgcccgcgcgggaccagcagcgcgaactttttgccgctcggccagcctggcaggggattttaaaatcggccaatcacagcgggcgccaggcctccgctttccgcttactggtcctgccgtaggaggcgggtacgtgagcgcaccaatctgtggccggcgagcgtaaagggcggggctccgcccaggctgcaccgcccagagcgcgcgt

SEQ ID NO: 16025 - RNA, 2359 nt, Homo sapiens
  source 1..2359: mol_type = other RNA
gctgggattacaggcatgagccatgcacccctacttctttagtgggagtctgtgccacagctgtggacacaggtgtccctagttattaaattagactttgtggtattttccccatcaggatgttcacacttccatgtggctaaagctattgatcttttctgttctggctcctgagctgagattttcttaaactctttctggatgaaatctttatttcatcaggctggtggcgtccacggcctcaactttacctccgtgatggaagagggggatctgaggctcccaggtgggccggcgccgccctacaggaaaggaggggtccctgggaggggctgttgccctggtggggttcacaggcccctcactgcaggggacccggagcaagggatgccccctggaatggccccgtgaccagaaagcgagcctgcccagcttccccaggaggagcctgcagtccacactcgcgtagccactccgggtggtggcagggtctctccctgctcccttccatagtcccgccacagcccacagccctgaggaagcctgggggtggagggtgccccggccagggtctctgtgactcacactcagggtgggccaggcgtccacaggctgggggcgggctggaggacagtggcagccccaggtggccacacagcatggtggtggtggtggtggtggtgcacggcaggcagccttggcctggcagctcgtgggaccctcgggggcacatgtggcgggtcctgcagggctgggggcagggccttgagcatccagttctgcaggaccaactggtgcacctgtgcgttctgcagcagcagcagctccaccatgtcttccttaatacttcctgaccgttgagtagggaaggcctggggaggaggaatctgtgctatgagtggctgctgagggagctgctgaatgatggtggcaggaggctgggggaccgtaggcaggatgatccttggcgggtctggggccagcggggatggggaggcagtgggtaggatgcccgtggggggcagctctgggggcagggctgacccgagggctcctctgcttggcccgctccaggcctgggcccgagagagctcgtccaggaggtgttgttcctgcaaggccgatgcagagctgctgcacacggggacggggagccccaacgccacagaggcacccccagcatcaggctcaggccagcctgggccaggtacaggcgcctctccgggcaggatggccatgactggaagacccttccagggttatgtgcatgagggtggcctcccggagtctctgcagaaggtccctccttctcttcagagcagtctgcagggcatcgtccggccggtcctcatttcctggctcgaggtggaggccctcaggtcccccttccacgttctgccgttcttgctccagcttctgtcccaagagcttcagcgtcagtcgggtcacttgctctgctgctgatgagtccagcatggtgggagctgcaggagacgactgtaggggcaggggaggccacagcccacctccctccctggttctgttactcgcaggaaagaactgctcagcaggagcccaagcaccggtgttgcctgcagggcgggccttacctcctggagaccagcgcgcgcgccagctgagaaaacgcccaccccggcggtcccgccacaggtcacaggcggtgcggaccccgggactgtgtccgggcttcggtgtccagagagctccaagacacccaaaccttccgtggtttccacctctgcaagcttatgttccgctgagctcaagctgagggacgacgacctcatgcgacgtcagtttccccctgggaccacgaacccacggccccatttctcttctgtctactaaaaaccttttcttttcttttttttttgagacctaagacatcagtgagacacacgagcagacacgggctcggtcgggaaaggcgggagctccaagcggcggggcctgcaggtccaggcggttcgcgggctttctgaccgcattcggccgagttcttctctgaagacccaggacccccggccgagggggcgcattcggcgggctggtggcgtaggattttgtttcgggttcccagggtcccggcaagggtgagggagcccttgcggatcccctgagatccacctcagcagcctcctccgtggtaggcctcaacttcccgcggcggcccacagccaacgactaatgcctgagcgggagaaaacggcctggccctgtccgggtggttgctgagcaccgttcggcgccgcccgcgcctgcagggagcccggcccgctgtcctggtggacacaaagcccaggggccgcccgcgcgggaccagcagcgcgaacttttt

SEQ ID NO: 16026 - RNA, 1706 nt, Homo sapiens
  source 1..1706: mol_type = other RNA
gctgggattacaggcatgagccatgcacccctacttctttagtgggagtctgtgccacagctgtggcacacaggtgtccctagttattaaattagactttgtggtattttccccatcaggatgttcacacttccatgtggctaaagctattgatcttttctgttctggctcctgagctgagattttcttaaactctttctggatgaaatctttatttcatcaggctggtggcgtccacggcctcaactttacctccgtgatggaagagggggatctgaggctcccaggtgggccggcgccgccctacaggaaaggaggggtccctgggaggggctgttgccctggtggggttcacaggcccctcactgcaggggacccggagcaagggatgccccctggaatggccccgtgaccagaaagcgagcctgcccagcttccccaggaggagcctgcagtccacactcgcgtagccactccgggtggtggcagggtctctccctgctcccttccatagtcccgccacagcccacagccctgaggaagcctgggggtggagggtgccccggccagggtctctgtgactcacactcagggtgggccaggcgtccacaggctgggggcgggctggaggacagtggcagccccaggtggccacacagcatggtggtggtggtggtggtggtgcacggcaggcagccttggcctggcagctcgtgggaccctcgggggcacatgtggcgggtcctgcagggctgggggcagggccttgagcatccagttctgcaggaccaactggtgcacctgtgcgttctgcagcagcagcagctccaccatgtcttccttaatacttcctgaccgttgagtagggaaggcctggggaggaggaatctgtgctatgagtggctgctgagggagctgctgaatgatggtggcaggaggctgggggaccgtaggcaggatgatccttggcgggtctggggccagcggggatggggaggcagtgggtaggatgcccgtggggggcagctctgggggcagggctgacccgagggctcctctgcttggcccgctccaggcctgggcccgagagagctcgtccaggaggtgttgttcctgcaaggccgatgcagagctgctgcacacggggacggggagccccaacgccacagaggcacccccagcatcaggctcaggccagcctgggccaggtacaggcgcctctccgggcaggatggccatgactggaagacccttccagggttatgtgcatgagggtggcctcccggagtctctgcagaaggtccctccttctcttcagagcagtctgcagggcatcgtccggccggtcctcatttcctggctcgaggtggaggccctcaggtcccccttccacgttctgccgttcttgctccagcttctgtgaggaagagagaccgtgacagagacggtggctccacgcaaaggccctgtgtgctccaggaatgactaagaggctttctgtcccaagagcttcagcgtcagtcgggtcacttgctctgctgctgatgagtccagcatggtgggagctgcaggagacgactgtaggggcaggggaggccacagcccacctccctccctggttctgttactcgcaggaaagaactgctcagcaggagcccaagcaccggtgttgcctgcagggcgggccttacctcctggagaccagc

SEQ ID NO: 16027 - RNA, 6626 nt, Homo sapiens
  source 1..6626: mol_type = other RNA
gctgggattacaggcatgagccatggcaccacctggccacttttttttttttttttttttgagacagtctcgttctgtcacccaggctggagtgcagtggtgcgatcttagctcactgcaacctctgcctcccaggttcaaccaattctcctgcctcagcctcctgagtagctgggattacaggtgccagccaccatgcccagctaatttttgtattttgggtagagatggggtttctttttttttttttggagacagagtctcactctgtcacccaggatagagtgcagtggcgcgatctcggctcactgcaagctccgcctcctgggttcacaccattctcctgccttagcctcccgatcagctgggactacaggcgcccaccaccacgcctggctaattttttgtatttttagtagagacggggtttcaccgtgttagccaggatggtctcgatctcctgacctcgtgatccacccgcctcagcctcccaaagtgctgggattacaggcgtgagccaccgcgcccggccgagatgggatttcaccatgttggccaggctagtctcgaactcttgacctcatgtgatccgcccacctcggcctcccaaagtgctgggattacgggtgtgagccactgcacctggcctgaatttgttgtttttaagtgagcaatttggttgcatttagtaaattcacaatgttgtacaaccaccacctgtatctggttccaaaacattttcatcaccccaaaagggcaccccaccattagaagtcactcccccttggtcccttcccagggcccccagcaatcgaccttctctctatatagatttgcctgttctggatatttcctataagtgaaatcatacagtccttctccttttgtgtctggcttctttcactcagcatcatgttttcaaggttcatccacatcgcaacatgcatcagcacttccttcctttttatggctaaataatattccactgcatggatatgtcacattttgtctgtccattcatctattgactgatatttgggttgattccatctctgagctgtcgtgaatagtgctgctgtgaacgtccgtgtacaagtttttgttgggagtctctgttttcaattctttccagtatgtgatcctggtctttgattccctcattacactgcctgccaaatgtacagccaaattgtatgcaacatcgttggaaggacaccggtgggaggggctgtcctgttaattcttggagaaatagcgtcgtagttcaatgtatgtcccacaaggtggcgcccacacttaggaagcttctccgggctgaaggaaaagctctctgtgccctctgtgcagccacaagtggaggctctacccagaagcagcggctttacacctaatactcctgtgactgacccacatccgaatacccagggagattaggtggttcatcacctgagagctttgtttttacttcagacagctgcttaaggttctaatgggttcctgtcactaaaagtgcaaggagattaatgtgtctaggttgtcaaaatcaacttgatagacatttcttcatagctaatatttcctttcttatctgttggttaaaagagccgatcctctcacagttacagtgagtacagcaggaaagaaatattacatttctctactttttccaattcacccctaccaaggttctttgcagtattcttttcttgttttttgtgtttttttcagagatggggtctcactctgggctggagtgaagtggtgcaatcacagctcactgcagccttgacctcctgggctcaagtgatcctcccacatcagcctccagagtaactgggaccacaggcacacatcaccacgctcagctaatttttgtatttttttgtagagatggggtttcaccatattggccaggctgatcttgaactcgtgggctgaagcaaatcacccacctcagcttcccaaaatgctgggattacaggcatgagccacagtgcctggcctaaaatactcttaaatgatgcaccctccatacatagaaaatcttcctagaagtaatatcatcctatataatgagatgagggttaagctggtgataaagttaggcataagtagggcatcaccctaaatcccgagttaagaggagtttgctgtagtttggggagcatattgaaaacacattgttggctgtgggcggcaagccatccaggtgctgaggcaagagaccgagggcacgagctgttccagtataataaaatatataaaacaacaagagttatactagatctagatcacagacatgattatatatgaatatcattaatcattagttatccggaggcctaaccgtctccctgtggtgctgtgcttcagtggtcacgctcctagtctgccttcatgttccatcctgtacacctggctctgccttttagataacagtagcaaaattagtgaaagtactaaaagtctctgatacgcagaaataatggcgtaagctgtctctctctctccctgtctatctctgccttggctgccaggcagggaagggccccctgtccagtggacacgtgacccacgtgaccttacctgtcattggagatgactcacactctttaccctgccccttttgctttgtatccaataaataacagtgcagccagacattcggggcctctaccggtctccgcctcttggtggtagtggtcccccaagcccagctgtcttttcttttacctctttgtcttgtgtctttatttctacaatctctcgtctccgcacatggggagaaaaacccaccgaccctgtggggctggtccctacagttggccgggcacggtggctcacacttgtaatcccagtactctgggaggcagaggtgggtggattacctgaggtcaggccttcaacaccagcctggccaacatggcaaaaccccgtctctactaaaaatacaaaaattagccaggcatggtggcgcacacctgtaatcccagctactcaggaggctgaggcaggagaattgctccaacccaggaggcagaggttgcagtgagccaagatcacgtcactgcactccagcctgggcgacagaccgagactcagtctcaaaaaaaaaagaagaaaaaaaaaaagaaaatacattgtcaagactcaaatcacagagtggtgtttcacatgatggtagagactgctgattgccctcttgaacccagcttccatttcttctttttcttatttatttatattttgagacggagtttctctcttgttgcccaggctggagtacaatggagcaatcttggctcactgcaacctctgcctcccaggttcaagcaattctcctgcctcagcctcctgagtagctgggattacaggcatgagccaccatgcccggctagtttttttttttttttttgtattttcagtagagatggggtttctccctgttggtcaggctggtctcgaactcccaacctcaggtgacccacccaccttggcctcccaaagtgctggaattataggcgtgagccactgtgcccggcctttgccaggtatcttgactagaggaagatagtgttctgggtgggagactcaagaggtctggttactgaagatacagatctcacttaaagtaagtaaattgacatctggtttccaaatcaatctattatgaaattggcccatgtcactttcatttggcctgatcaagtttttactgagaactgaattgggcacagtggctcacacctgtaatcccagcaccttaggaggctaaggcgggaggatcacttgagtccaggagtttgaaaacagcctgggcaacataacaaagtcccatctccacaaaaaatacaaacattagcccaggaagctgaagcaggaggatcatttgagcccaggaggtcgaggcagcagtgagctatgatcgtgccactgcactccagcctggatggcagagcaagaccctgtctcaaaaaaaaaaaaaaaaaaaatttgagaacattggacattcagtatctctcccctctcttgggcatcatgtttaggttctgtctctagagcacatctcagagcctgctacaggtaaacaggccagaagttaaatgcatgaaacaaattaaatgcatgaaacattcaagcacattcttattggtgtaattaaaataaaaaagtaaatgcatgaaacagaagctgtttacccacagcagaggaggggcagaaatcatatccagtgtgccatatcattactgcctgccagcatttccttaggctatttcatttatttactttttttgagatggagtctcgctctgactcccaggctggagtgcagtggcatgatctccactcactgcaacctccacctcccaggttcaaccaattttcctgcctcagcctcccaagtagctgggattacaggtgccagccaccatgactgcctaatttgtgtatttttagtgagagacagggtttcactacgttggccaggctggtctcaaactcctgacctcgagtgatccacccgcctcggcttcccaaagtgctgggattacaggcgtgagccaccatgcccaccttcctttggttattgagatggacaaagagttacccagtaagttaagagcagctagtttttaatgaatcttagcccagaatacaaagcagggtgtagcagttgccttaatggtgatataattgtaaacaatagctttttcttcccctataaactcgagttataggaagcgtttcagagagaggataacacatttgaatctattttttaaaaatcatcctgaaagctagcagtattgttgtcgtttaaaaggttcctcatatactcttaccctcagccaacccaccatgtttatcaattcaaattctagaactttcttgacccaagagattttgtaggaaaaatttctcttttcagatattcagcacgcaaggatcatttttcttggttttgttgctgatcttgctgaactttccatcaatggctgagggaggaagcttgcatgattcttatgagttcttctgaggcactttgactgtgacagttttcacttcagtgtatgcctgcagcccgtactcgcccaactcccggccactccccgacatcttgtagccaccaaagggtgactgggctccaaacacatcatagcagttgacccacacagtgcccgcctggagggcctgggacaggtaattggccttgtccaaatcctttgtgaagacagctgcggccagcccgtacgtggaattgttggctctcccaacaacctcctctatggtcttgaacttcaggatctgcatcactggcccgaagatctcctccttggcgatggtcatgccatcctgcacatctccaaacacagtgggctggatgaagtaaccacggtcagcagcaatgcccccaccacacagcagcttcgccccctcttgcttccccgtgttgatgtagccgaggatcttcttaaactgagtttcatccacctgcggcccctgctcggtcttgctatcaaaggggttcccgaccacccgagacttggcccgggcaacgctccgctccacaaactcatcatagatgtcctcctgcacgaaggtccgggagccggcacagcagcactggccctggttgaagaacagggcgaagtgggcctgttccacggcccaatccatatcggcatctgacatgatgatgttggggctcttcccccccagctccaaggtcactctcttgaggttgctgctcccagcagcaacctggattacgcggccaatctcagtggagcctgtgaatgccactttgtccacatcctcatgggaggcaatggcggccccagccgtggggccaaatccaggcacaatgttgaccacaccagggggaaagccagcctccttgatcaggttggccacatagagggcggtgaggggtgtctgctcagctaccttcatcacaaccacgtttccagttgccaaggctgggcccagcttccatgcttgcatcaggagcgggaaattccacggaatgatctgcccgcacacccccacaggttcatggcgtgtgtagctgaagaagtctccgtcaatggggatggttttcccgtggtacttatcagcccagccggcataataccggagacatttgaggaccatgtccaaatccaccaggtaggagatgacatagggcttgccattgtccagggtctccaaggccgccaggtaggtccggtcccgctcgatcagatcggccaggcggttcagcagccggcccctgtgtgatgcgtccatgcggcgccaaggtgagcccagctggaaggcggcccgggcggccttcactgccttgtccacatcttccttgtccccttcagctacctgacagatgacctctccagtggacggattgacggtggggaatgttttcctgctgacggcatcgtgccattcattgtttatgaaaatctggttgcagaagacctcgggctgctggttgggggcaggcacggcctgggtggcggcggctgacaagaggcggcggcccaggcggggcccgaagcgggcggcagcgcgcaacatcgcagcgggctagcggacagcgagcggaccgagagcagagctagggtctc

SEQ ID NO: 16028 - RNA, 6485 nt, Homo sapiens
  source 1..6485: mol_type = other RNA
gctgggattacaggcatgagccatggcaccacctggccacttttttttttttttttttttgagacagtctcgttctgtcacccaggctggagtgcagtggtgcgatcttagctcactgcaacctctgcctcccaggttcaaccaattctcctgcctcagcctcctgagtagctgggattacaggtgccagccaccatgcccagctaatttttgtattttgggtagagatggggtttctttttttttttttggagacagagtctcactctgtcacccaggatagagtgcagtggcgcgatctcggctcactgcaagctccgcctcctgggttcacaccattctcctgccttagcctcccgatcagctgggactacaggcgcccaccaccacgcctggctaattttttgtatttttagtagagacggggtttcaccgtgttagccaggatggtctcgatctcctgacctcgtgatccacccgcctcagcctcccaaagtgctgggattacaggcgtgagccaccgcgcccggccgagatgggatttcaccatgttggccaggctagtctcgaactcttgacctcatgtgatccgcccacctcggcctcccaaagtgctgggattacgggtgtgagccactgcacctggcctgaatttgttgtttttaagtgagcaatttggttgcatttagtaaattcacaatgttgtacaaccaccacctgtatctggttccaaaacattttcatcaccccaaaagggcaccccaccattagaagtcactcccccttggtcccttcccagggcccccagcaatcgaccttctctctatatagatttgcctgttctggatatttcctataagtgaaatcatacagtccttctccttttgtgtctggcttctttcactcagcatcatgttttcaaggttcatccacatcgcaacatgcatcagcacttccttcctttttatggctaaataatattccactgcatggatatgtcacattttgtctgtccattcatctattgactgatatttgggttgattccatctctgagctgtcgtgaatagtgctgctgtgaacgtccgtgtacaagtttttgttgggagtctctgttttcaattctttccagtatgtgatcctggtctttgattccctcattacactgcctgccaaatgtacagccaaattgtatgcaacatcgttggaaggacaccggtgggaggggctgtcctgttaattcttggagaaatagcgtcgtagttcaatgtatgtcccacaaggtggcgcccacacttaggaagcttctccgggctgaaggaaaagctctctgtgccctctgtgcagccacaagtggaggctctacccagaagcagcggctttacacctaatactcctgtgactgacccacatccgaatacccagggagattaggtggttcatcacctgagagctttgtttttacttcagacagctgcttaaggttctaatgggttcctgtcactaaaagtgcaaggagattaatgtgtctaggttgtcaaaatcaacttgatagacatttcttcatagctaatatttcctttcttatctgttggttaaaagagccgatcctctcacagttacagtgagtacagcaggaaagaaatattacatttctctactttttccaattcacccctaccaaggttctttgcagtattcttttcttgttttttgtgtttttttcagagatggggtctcactctgggctggagtgaagtggtgcaatcacagctcactgcagccttgacctcctgggctcaagtgatcctcccacatcagcctccagagtaactgggaccacaggcacacatcaccacgctcagctaatttttgtatttttttgtagagatggggtttcaccatattggccaggctgatcttgaactcgtgggctgaagcaaatcacccacctcagcttcccaaaatgctgggattacaggcatgagccacagtgcctggcctaaaatactcttaaatgatgcaccctccatacatagaaaatcttcctagaagtaatatcatcctatataatgagatgagggttaagctggtgataaagttaggcataagtagggcatcaccctaaatcccgagttaagaggagtttgctgtagtttggggagcatattgaaaacacattgttggctgtgggcggcaagccatccaggtgctgaggcaagagaccgagggcacgagctgttccagtataataaaatatataaaacaacaagagttatactagatctagatcacagacatgattatatatgaatatcattaatcattagttatccggaggcctaaccgtctccctgtggtgctgtgcttcagtggtcacgctcctagtctgccttcatgttccatcctgtacacctggctctgccttttagataacagtagcaaaattagtgaaagtactaaaagtctctgatacgcagaaataatggcgtaagctgtctctctctctccctgtctatctctgccttggctgccaggcagggaagggccccctgtccagtggacacgtgacccacgtgaccttacctgtcattggagatgactcacactctttaccctgccccttttgctttgtatccaataaataacagtgcagccagacattcggggcctctaccggtctccgcctcttggtggtagtggtcccccaagcccagctgtcttttcttttacctctttgtcttgtgtctttatttctacaatctctcgtctccgcacatggggagaaaaacccaccgaccctgtggggctggtccctacagttggccgggcacggtggctcacacttgtaatcccagtactctgggaggcagaggtgggtggattacctgaggtcaggccttcaacaccagcctggccaacatggcaaaaccccgtctctactaaaaatacaaaaattagccaggcatggtggcgcacacctgtaatcccagctactcaggaggctgaggcaggagaattgctccaacccaggaggcagaggttgcagtgagccaagatcacgtcactgcactccagcctgggcgacagaccgagactcagtctcaaaaaaaaaagaagaaaaaaaaaaagaaaatacattgtcaagactcaaatcacagagtggtgtttcacatgatggtagagactgctgattgccctcttgaacccagcttccatttcttctttttcttatttatttatattttgagacggagtttctctcttgttgcccaggctggagtacaatggagcaatcttggctcactgcaacctctgcctcccaggttcaagcaattctcctgcctcagcctcctgagtagctgggattacaggcatgagccaccatgcccggctagtttttttttttttttttgtattttcagtagagatggggtttctccctgttggtcaggctggtctcgaactcccaacctcaggtgacccacccaccttggcctcccaaagtgctggaattataggcgtgagccactgtgcccggcctttgccaggtatcttgactagaggaagatagtgttctgggtgggagactcaagaggtctggttactgaagatacagatctcacttaaagtaagtaaattgacatctggtttccaaatcaatctattatgaaattggcccatgtcactttcatttggcctgatcaagtttttactgagaactgaattgggcacagtggctcacacctgtaatcccagcaccttaggaggctaaggcgggaggatcacttgagtccaggagtttgaaaacagcctgggcaacataacaaagtcccatctccacaaaaaatacaaacattagcccaggaagctgaagcaggaggatcatttgagcccaggaggtcgaggcagcagtgagctatgatcgtgccactgcactccagcctggatggcagagcaagaccctgtctcaaaaaaaaaaaaaaaaaaaatttgagaacattggacattcagtatctctcccctctcttgggcatcatgtttaggttctgtctctagagcacatctcagagcctgctacaggtaaacaggccagaagttaaatgcatgaaacaaattaaatgcatgaaacattcaagcacattcttattggtgtaattaaaataaaaaagtaaatgcatgaaacagaagctgtttacccacagcagaggaggggcagaaatcatatccagtgtgccatatcattactgcctgccagcatttccttaggctatttcatttatttactttttttgagatggagtctcgctctgactcccaggctggagtgcagtggcatgatctccactcactgcaacctccacctcccaggttcaaccaattttcctgcctcagcctcccaagtagctgggattacaggtgccagccaccatgactgcctaatttgtgtatttttagtgagagacagggtttcactacgttggccaggctggtctcaaactcctgacctcgagtgatccacccgcctcggcttcccaaagtgctgggattacaggcgtgagccaccatgcccaccttcctttggttattgagatggacaaagagttacccagtaagttaagagcagctagtttttaatgaatcttagcccagaatacaaagcagggtgtagcagttgccttaatggtgatataattgtaaacaatagctttttcttcccctataaactcgagttataggaagcgtttcagagagaggataacacatttgaatctattttttaaaaatcatcctgaaagctagcagtattgttgtcgtttaaaaggttcctcatatactcttaccctcagccaacccaccatgtttatcaattcaaattctagaactttcttgacccaagagattttgtaggaaaaatttctcttttcagatattcagcacgcaaggatcatttttcttggttttgttgctgatcttgctgaactttccatcaatggctgagggaggaagcttgcatgattcttatgagttcttctgaggcactttgactgtgacagttttcacttcagtgtatgcctgcagcccgtactcgcccaactcccggccactccccgacatcttgtagccaccaaagggtgactgggctccaaacacatcatagcagttgacccacacagtgcccgcctggagggcctgggacaggtaattggccttgtccaaatcctttgtgaagacagctgcggccagcccgtacgtggaattgttggctctcccaacaacctcctctatggtcttgaacttcaggatctgcatcactggcccgaagatctcctccttggcgatggtcatgccatcctgcacatctccaaacacagtgggctggatgaagtaaccacggtcagcagcaatgcccccaccacacagcagcttcgccccctcttgcttccccgtgttgatgtagccgaggatcttcttaaactgagtttcatccacctgcggcccctgctcggtcttgctatcaaaggggttcccgaccacccgagacttggcccgggcaacgctccgctccacaaactcatcatagatgtcctcctgcacgaaggtccgggagccggcacagcagcactggccctggttgaagaacagggcgaagtgggcctgttccacggcccaatccatatcggcatctgacatgatgatgttggggctcttcccccccagctccaaggtcactctcttgaggttgctgctcccagcagcaacctggattacgcggccaatctcagtggagcctgtgaatgccactttgtccacatcctcatgggaggcaatggcggccccagccgtggggccaaatccaggcacaatgttgaccacaccagggggaaagccagcctccttgatcaggttggccacatagagggcggtgaggggtgtctgctcagctaccttcatcacaaccacgtttccagttgccaaggctgggcccagcttccatgcttgcatcaggagcgggaaattccacggaatgatctgcccgcacacccccacaggttcatggcgtgtgtagctgaagaagtctccgtcaatggggatggttttcccgtggtacttatcagcccagccggcataataccggagacatttgaggaccatgtccaaatccaccaggtaggagatgacatagggcttgccattgtccagggtctccaaggccttgtccccttcagctacctgacagatgacctctccagtggacggattgacggtggggaatgttttcctgctgacggcatcgtgccattcattgtttatgaaaatctggttgcagaagacctcgggctgctggttgggggcaggcacggcctgggtggcggcggctgacaagaggcggcggcccaggcggggcccgaagcgggcggcagcgcgcaacatcgcagcgggctagcggacagcgagcggaccgagagcagagctagggtctc

SEQ ID NO: 16029 - RNA, 3513 nt, Homo sapiens
  source 1..3513: mol_type = other RNA
gctgggattacaggcatgagccatggcacctgacccaccattacttttattttgaatcttgtctgtgtagcaagcagtgcagtgagaaattttgttggcagaggaaaaaaattcctttttgcatcaggtcaagcccccaaactagccaaagaaaagctgtgtaatctattcagaagtactggagatgtgctgcacattagggagaatggagaattactggtcacaacgaatcccggtttctatcacccatagctatgtgaacccagacaatcattaagcaatctgggttggttagatggcttctaagatctctttcaataaaaaagttctaagattcagaattcctgagaagttgcagctaacatacactgtataagattttatacattaaaaacaaacatctcatttggtcttaacccagtaggaagaaaagattaaaatattttgtatttgaaataaacagaccctaatattaattatgaccagggaaataattttaaaacatcccaaaggaaagttctctaacttttaaaatattataaattaatactgcaacaggagctacctcaaatctctcaacaaagatggaatataattaaatagaagaactagcaccagttatcaactatgtgcctgcccttgaactctctgcatttttgtagttctgttttaaagatgaggaaaataagcttcatagataaatgttattttgtctaaggtcatccagtttgcttctccattaaacaatcaattaagatgactattcagtgcacaaactgtaatctgttttattaatacttccaagttttctacatgactctggatttatactttgtatcaattctcttgctggttaagaaaaaaaacaagatttattaaaaactgaccataaataatgtgtaaactaaggagagttttgtctttttccttactgaaggacaaggaatcagtaaagaagttctttgctttgcttaatgaagatcaaaacctggtaattaaatttggctaatataatcattccttttctgacaagacttttttcacctttattcacctgagtaacttacctgtttccaaagacacctaggaaattcagaatgttatatatgcttttccttatttactataatttataggacatgagtggatggattctcttcaatagagaaaatgattttctctaattaaaatgcaccaaattgatgtactaagagattgctttagatgaacacatttatgttcagtgaagattatgtggtcttcaatgacactgcaatataattactaggtacaaaacaaaagcagagatccacacacaatggctcactgtcttcgatgacaacacttttaggatctcatttattcattctttaagtaatttttcttttaaaaaagggataggtggaaaaaatagttgggaaatctttaactaggctaaggtttagacataggtataaattatttattttgtaacattcaaaaaccaaaaaccaccctgacatactgggtggcaagaaaagtcaagatcagattaaacatttgttttgcactaatcacaaaactaataatccaagtcactatcatcaactccagttgatctcagctctgattatgcatcagaacaccctgtgaggtctattaagttcctataccaaatcccaaacactcttgaatcagtctacaaagttgggacctaggtatctgtacattttttaaagttcctcaaaaaattctgcttctaggcaaatgtaatagatattgtgcgttgctcatgtttttcctatcagaaccatgattttaaaaaaactatcctttctgtccccatatatccctcatgtggcctccacttctactctcagctccagtggacctgactgccctaaaggttattctagaccctttgccagtgactggctcagggatggacaggtctaagttactttagagcaatgagacctaaggatatggaaagtgaattctgggaaagctttctcatactaggacagggcccctagaatccagcctgactcttccgctgcatgtaaatgaagatgcacaaggctccaactgctactggcaatcatcccatgaccacgagggtagccagccttaggatgatgccaatgttgtggttgaaaagggggtggggtgtggaggcgggttcccaaggttcttgatgacattactgaatcattggatcagaaacactgcagcacattctgtcaatagatttcatgtattgtgaatcaatatattttcttactgtttttaagtcattttaagttggacttttagtggtcagcatctgaatgttaaagagtggtcccagcacagcattctttaattataacaatctgtatcaagtagaatccacacaaacaccccttcgtacttacataatctgtaaatctgatgtatctttcctattttaacaaaatctttaatttatatcgttataccttactaaagtgttaatgtgcattgcattcacttcattatttactcagagttcttgctgtaggctttgtcttgaatgtgtaggaccattcgtcgtgcatagaagtccctatattcctctggtaactcggccagtgttttcaaggctctgtccagaatttgtgcagctcttgatgctgctgtaggatctttgtttccataggtatctgttttatcatagcattcagatggaaggtgcttccaaaagatattcactcccactccaaactcttcagaaattacattatggaaccataaagcaggaatgaataatacatcaccagcttcaagggaacattcatatcttctagccttggaaaaaagtggatatttagccaagtctgggttatctatattcagtacttctgatttagtacatcataatgagtccatagttgtaatcctggtgaactaattcgaaaaacactggaaaagaactgttcctctttgaagaattctggaaacttaatatctcctttcaacaaaggaaactgctttctgatatctgcaacatcctttctagggtcttctccaagtgaccgtaagtagtatttctcatcctctgaaacaaagaattctttatgtttctcttcagctgccctctggaccaactggtcaaaaggtaaagttctatatacaaagttcttactaatgaagtccatctgtgcaactgcagcaacatgaatctttacttctttcttccctccaacttggcttaggtaatccactgtccatttgcttgtacatggccccaaatcaatcccttccaacacaagaggttttctctgtgggtagaggtgctgcatgaactgctcccgagaaacgccctccagccggggtaccgggaggtgctgcccggccatggttgctcacgcctgccctcttccaggtcttcggaacttcggctctaaagcgttcctcagcgccatccgcccggaaacacgagcgacagagaaaaggtccgcgaggccggcagactccagagtggctgggtccgagcgcggggcgggttgccga

SEQ ID NO: 16030 - RNA, 3361 nt, Homo sapiens
  source 1..3361: mol_type = other RNA
gctgggattacaggcatgagccatggcacctgacccaccattacttttattttgaatcttgtctgtgtagcaagcagtgcagtgagaaattttgttggcagaggaaaaaaattcctttttgcatcaggtcaagcccccaaactagccaaagaaaagctgtgtaatctattcagaagtactggagatgtgctgcacattagggagaatggagaattactggtcacaacgaatcccggtttctatcacccatagctatgtgaacccagacaatcattaagcaatctgggttggttagatggcttctaagatctctttcaataaaaaagttctaagattcagaattcctgagaagttgcagctaacatacactgtataagattttatacattaaaaacaaacatctcatttggtcttaacccagtaggaagaaaagattaaaatattttgtatttgaaataaacagaccctaatattaattatgaccagggaaataattttaaaacatcccaaaggaaagttctctaacttttaaaatattataaattaatactgcaacaggagctacctcaaatctctcaacaaagatggaatataattaaatagaagaactagcaccagttatcaactatgtgcctgcccttgaactctctgcatttttgtagttctgttttaaagatgaggaaaataagcttcatagataaatgttattttgtctaaggtcatccagtttgcttctccattaaacaatcaattaagatgactattcagtgcacaaactgtaatctgttttattaatacttccaagttttctacatgactctggatttatactttgtatcaattctcttgctggttaagaaaaaaaacaagatttattaaaaactgaccataaataatgtgtaaactaaggagagttttgtctttttccttactgaaggacaaggaatcagtaaagaagttctttgctttgcttaatgaagatcaaaacctggtaattaaatttggctaatataatcattccttttctgacaagacttttttcacctttattcacctgagtaacttacctgtttccaaagacacctaggaaattcagaatgttatatatgcttttccttatttactataatttataggacatgagtggatggattctcttcaatagagaaaatgattttctctaattaaaatgcaccaaattgatgtactaagagattgctttagatgaacacatttatgttcagtgaagattatgtggtcttcaatgacactgcaatataattactaggtacaaaacaaaagcagagatccacacacaatggctcactgtcttcgatgacaacacttttaggatctcatttattcattctttaagtaatttttcttttaaaaaagggataggtggaaaaaatagttgggaaatctttaactaggctaaggtttagacataggtataaattatttattttgtaacattcaaaaaccaaaaaccaccctgacatactgggtggcaagaaaagtcaagatcagattaaacatttgttttgcactaatcacaaaactaataatccaagtcactatcatcaactccagttgatctcagctctgattatgcatcagaacaccctgtgaggtctattaagttcctataccaaatcccaaacactcttgaatcagtctacaaagttgggacctaggtatctgtacattttttaaagttcctcaaaaaattctgcttctaggcaaatgtaatagatattgtgcgttgctcatgtttttcctatcagaaccatgattttaaaaaaactatcctttctgtccccatatatccctcatgtggcctccacttctactctcagctccagtggacctgactgccctaaaggttattctagaccctttgccagtgactggctcagggatggacaggtctaagttactttagagcaatgagacctaaggatatggaaagtgaattctgggaaagctttctcatactaggacagggcccctagaatccagcctgactcttccgctgcatgtaaatgaagatgcacaaggctccaactgctactggcaatcatcccatgaccacgagggtagccagccttaggatgatgccaatgttgtggttgaaaagggggtggggtgtggaggcgggttcccaaggttcttgatgacattactgaatcattggatcagaaacactgcagcacattctgtcaatagatttcatgtattgtgaatcaatatattttcttactgtttttaagtcattttaagttggacttttagtggtcagcatctgaatgttaaagagtggtcccagcacagcattctttaattataacaatctgtatcaagtagaatccacacaaacaccccttcgtacttacataatctgtaaatctgatgtatctttcctattttaacaaaatctttaatttatatcgttataccttactaaagtgttaatgtgcattgcattcacttcattatttactcagagttcttgctgtaggctttgtcttgaatgtgtaggaccattcgtcgtgcatagaagtccctatattcctctggtaactcggccagtgttttcaaggctctgtccagaatttgtgcagctcttgatgctgctgtaggatctttgtttccataggtatctgttttatcatagcattcagatggaaggtgcttccaaaagatattcactcccactccaaactcttcagaaattacattatggaaccataaagcaggaatgaataatacatcaccagcttcaagggaacattcatatcttctagccttggaaaaaagtggatatttagccaagtctgggttatctatattcagtacttctgatttagtacatcataatgagtccatagttgtaatcctggtgaactaattcgaaaaacactggaaaagaactgttcctctttgaagaattctggaaacttaatatctcctttcaacaaaggaaactgctttctgatatctgcaacatcctttctagggtcttctccaagtgaccgtaagtagtatttctcatcctctgaaacaaagaattctttatgtttctcttcagctgccctctggaccaactggtcaaaaggtaaagtttaatgaagtccatctgtgcaactgcagcaacatgaatctttacttctttcttccctccaacttggcttaggtaatccactgtccatttgcttgtacatggccccaaatcaatcccttccaacacaagaggttttctctgtgggtagaggtgctgcatgaactgctcccgagaaacgccctccagccggggtaccgggaggtgctgcccggccatggttgctcacgcctgccctct

SEQ ID NO: 16031 - RNA, 3197 nt, Homo sapiens
  source 1..3197: mol_type = other RNA
gctgggattacaggcatgagccatggcacctgacccaccattacttttattttgaatcttgtctgtgtagcaagcagtgcagtgagaaattttgttggcagaggaaaaaaattcctttttgcatcaggtcaagcccccaaactagccaaagaaaagctgtgtaatctattcagaagtactggagatgtgctgcacattagggagaatggagaattactggtcacaacgaatcccggtttctatcacccatagctatgtgaacccagacaatcattaagcaatctgggttggttagatggcttctaagatctctttcaataaaaaagttctaagattcagaattcctgagaagttgcagctaacatacactgtataagattttatacattaaaaacaaacatctcatttggtcttaacccagtaggaagaaaagattaaaatattttgtatttgaaataaacagaccctaatattaattatgaccagggaaataattttaaaacatcccaaaggaaagttctctaacttttaaaatattataaattaatactgcaacaggagctacctcaaatctctcaacaaagatggaatataattaaatagaagaactagcaccagttatcaactatgtgcctgcccttgaactctctgcatttttgtagttctgttttaaagatgaggaaaataagcttcatagataaatgttattttgtctaaggtcatccagtttgcttctccattaaacaatcaattaagatgactattcagtgcacaaactgtaatctgttttattaatacttccaagttttctacatgactctggatttatactttgtatcaattctcttgctggttaagaaaaaaaacaagatttattaaaaactgaccataaataatgtgtaaactaaggagagttttgtctttttccttactgaaggacaaggaatcagtaaagaagttctttgctttgcttaatgaagatcaaaacctggtaattaaatttggctaatataatcattccttttctgacaagacttttttcacctttattcacctgagtaacttacctgtttccaaagacacctaggaaattcagaatgttatatatgcttttccttatttactataatttataggacatgagtggatggattctcttcaatagagaaaatgattttctctaattaaaatgcaccaaattgatgtactaagagattgctttagatgaacacatttatgttcagtgaagattatgtggtcttcaatgacactgcaatataattactaggtacaaaacaaaagcagagatccacacacaatggctcactgtcttcgatgacaacacttttaggatctcatttattcattctttaagtaatttttcttttaaaaaagggataggtggaaaaaatagttgggaaatctttaactaggctaaggtttagacataggtataaattatttattttgtaacattcaaaaaccaaaaaccaccctgacatactgggtggcaagaaaagtcaagatcagattaaacatttgttttgcactaatcacaaaactaataatccaagtcactatcatcaactccagttgatctcagctctgattatgcatcagaacaccctgtgaggtctattaagttcctataccaaatcccaaacactcttgaatcagtctacaaagttgggacctaggtatctgtacattttttaaagttcctcaaaaaattctgcttctaggcaaatgtaatagatattgtgcgttgctcatgtttttcctatcagaaccatgattttaaaaaaactatcctttctgtccccatatatccctcatgtggcctccacttctactctcagctccagtggacctgactgccctaaaggttattctagaccctttgccagtgactggctcagggatggacaggtctaagttactttagagcaatgagacctaaggatatggaaagtgaattctgggaaagctttctcatactaggacagggcccctagaatccagcctgactcttccgctgcatgtaaatgaagatgcacaaggctccaactgctactggcaatcatcccatgaccacgagggtagccagccttaggatgatgccaatgttgtggttgaaaagggggtggggtgtggaggcgggttcccaaggttcttgatgacattactgaatcattggatcagaaacactgcagcacattctgtcaatagatttcatgtattgtgaatcaatatattttcttactgtttttaagtcattttaagttggacttttagtggtcagcatctgaatgttaaagagtggtcccagcacagcattctttaattataacaatctgtatcaagtagaatccacacaaacaccccttcgtacttacataatctgtaaatctgatgtatctttcctattttaacaaaatctttaatttatatcgttataccttactaaagtgttaatgtgcattgcattcacttcattatttactcagagttcttgctgtaggctttgtcttgaatgtgtaggaccattcgtcgtgcatagaagtccctatattcctctggtaactcggccagtgttttcaaggctctgtccagaatttgtgcagctcttgatgctgctgtaggatctttgtttccataggtatctgttttatcatagcattcagatggaaggtgcttccaaaagatattcactcccactccaaactcttcagaaattacattatggaaccataaagcaggaatgaataatacatcaccagcttcaagggaacattcatatcttctagccttggaaaaaagtggatatttagccaagtctgggttatctatattcagtacttctgatttagtacctctgaaacaaagaattctttatgtttctcttcagctgccctctggaccaactggtcaaaaggtaaagttctatatacaaagttcttactaatgaagtccatctgtgcaactgcagcaacatgaatctttacttctttcttccctccaacttggcttaggtaatccactgtccatttgcttgtacatggccccaaatcaatcccttccaacacaagaggttttctctgtgggtagaggtgctgcatgaactgctcccgagaaacgccctccagccggggtaccgggaggtgctgcccggccatggttgctcacgcctgccctct

SEQ ID NO: 16032 - RNA, 3468 nt, Homo sapiens
  source 1..3468: mol_type = other RNA
gctgggattacaggcatgagccatggcacctgacccaccattacttttattttgaatcttgtctgtgtagcaagcagtgcagtgagaaattttgttggcagaggaaaaaaattcctttttgcatcaggtcaagcccccaaactagccaaagaaaagctgtgtaatctattcagaagtactggagatgtgctgcacattagggagaatggagaattactggtcacaacgaatcccggtttctatcacccatagctatgtgaacccagacaatcattaagcaatctgggttggttagatggcttctaagatctctttcaataaaaaagttctaagattcagaattcctgagaagttgcagctaacatacactgtataagattttatacattaaaaacaaacatctcatttggtcttaacccagtaggaagaaaagattaaaatattttgtatttgaaataaacagaccctaatattaattatgaccagggaaataattttaaaacatcccaaaggaaagttctctaacttttaaaatattataaattaatactgcaacaggagctacctcaaatctctcaacaaagatggaatataattaaatagaagaactagcaccagttatcaactatgtgcctgcccttgaactctctgcatttttgtagttctgttttaaagatgaggaaaataagcttcatagataaatgttattttgtctaaggtcatccagtttgcttctccattaaacaatcaattaagatgactattcagtgcacaaactgtaatctgttttattaatacttccaagttttctacatgactctggatttatactttgtatcaattctcttgctggttaagaaaaaaaacaagatttattaaaaactgaccataaataatgtgtaaactaaggagagttttgtctttttccttactgaaggacaaggaatcagtaaagaagttctttgctttgcttaatgaagatcaaaacctggtaattaaatttggctaatataatcattccttttctgacaagacttttttcacctttattcacctgagtaacttacctgtttccaaagacacctaggaaattcagaatgttatatatgcttttccttatttactataatttataggacatgagtggatggattctcttcaatagagaaaatgattttctctaattaaaatgcaccaaattgatgtactaagagattgctttagatgaacacatttatgttcagtgaagattatgtggtcttcaatgacactgcaatataattactaggtacaaaacaaaagcagagatccacacacaatggctcactgtcttcgatgacaacacttttaggatctcatttattcattctttaagtaatttttcttttaaaaaagggataggtggaaaaaatagttgggaaatctttaactaggctaaggtttagacataggtataaattatttattttgtaacattcaaaaaccaaaaaccaccctgacatactgggtggcaagaaaagtcaagatcagattaaacatttgttttgcactaatcacaaaactaataatccaagtcactatcatcaactccagttgatctcagctctgattatgcatcagaacaccctgtgaggtctattaagttcctataccaaatcccaaacactcttgaatcagtctacaaagttgggacctaggtatctgtacattttttaaagttcctcaaaaaattctgcttctaggcaaatgtaatagatattgtgcgttgctcatgtttttcctatcagaaccatgattttaaaaaaactatcctttctgtccccatatatccctcatgtggcctccacttctactctcagctccagtggacctgactgccctaaaggttattctagaccctttgccagtgactggctcagggatggacaggtctaagttactttagagcaatgagacctaaggatatggaaagtgaattctgggaaagctttctcatactaggacagggcccctagaatccagcctgactcttccgctgcatgtaaatgaagatgcacaaggctccaactgctactggcaatcatcccatgaccacgagggtagccagccttaggatgatgccaatgttgtggttgaaaagggggtggggtgtggaggcgggttcccaaggttcttgatgacattactgaatcattggatcagaaacactgcagcacattctgtcaatagatttcatgtattgtgaatcaatatattttcttactgtttttaagtcattttaagttggacttttagtggtcagcatctgaatgttaaagagtggtcccagcacagcattctttaattataacaatctgtatcaagtagaatccacacaaacaccccttcgtacttacataatctgtaaatctgatgtatctttcctattttaacaaaatctttaatttatatcgttataccttactaaagtgttaatgtgcattgcattcacttcattatttactcagagttcttgctgtaggctttgtcttgaatgtgtaggaccattcgtcgtgcatagaagtccctatattcctctggtaactcggccagtgttttcaaggctctgtccagaatttgtgcagctcttgatgctgctgtaggatctttgtttccataggtatctgttttatcatagcattcagatggaaggtgcttccaaaagatattcactcccactccaaactcttcagaaattacattatggaaccataaagcaggaatgaataatacatcaccagcttcaagggaacattcatatcttctagccttggaaaaaagtggatatttagccaagtctgggttatctatattcagtacttctgatttagtaccttttaaatataaatactgggcatctcgaggactgaagagtacaacacgcttttttcctgtcacttgtattaacaaattatccattacatcataatgagtccatagttgtaatcctggtgaactaattcgaaaaacactggaaaagaactgttcctctttgaagaattctggaaacttaatatctcctttcaacaaaggaaactgctttctgatatctgcaacatcctttctagggtcttctccaagtgaccgtaagtagtatttctcatcctctgaaacaaagaattctttatgtttctcttcagctgccctctggaccaactggtcaaaaggtaaagttctatatacaaagttcttactaatgaagtccatctgtgcaactgcagcaacatgaatctttacttctttcttccctccaacttggcttaggtaatccactgtccatttgcttgtacatggccccaaatcaatcccttccaacacaagaggttttctctgtgggtagaggtgctgcatgaactgctcccgagaaacgccctccagccggggtaccgggaggtgctgcccggccatggttgctcacgcctgccctct

SEQ ID NO: 16033 - RNA, 3313 nt, Homo sapiens
  source 1..3313: mol_type = other RNA
gctgggattacaggcatgagccatggcacctgacccaccattacttttattttgaatcttgtctgtgtagcaagcagtgcagtgagaaattttgttggcagaggaaaaaaattcctttttgcatcaggtcaagcccccaaactagccaaagaaaagctgtgtaatctattcagaagtactggagatgtgctgcacattagggagaatggagaattactggtcacaacgaatcccggtttctatcacccatagctatgtgaacccagacaatcattaagcaatctgggttggttagatggcttctaagatctctttcaataaaaaagttctaagattcagaattcctgagaagttgcagctaacatacactgtataagattttatacattaaaaacaaacatctcatttggtcttaacccagtaggaagaaaagattaaaatattttgtatttgaaataaacagaccctaatattaattatgaccagggaaataattttaaaacatcccaaaggaaagttctctaacttttaaaatattataaattaatactgcaacaggagctacctcaaatctctcaacaaagatggaatataattaaatagaagaactagcaccagttatcaactatgtgcctgcccttgaactctctgcatttttgtagttctgttttaaagatgaggaaaataagcttcatagataaatgttattttgtctaaggtcatccagtttgcttctccattaaacaatcaattaagatgactattcagtgcacaaactgtaatctgttttattaatacttccaagttttctacatgactctggatttatactttgtatcaattctcttgctggttaagaaaaaaaacaagatttattaaaaactgaccataaataatgtgtaaactaaggagagttttgtctttttccttactgaaggacaaggaatcagtaaagaagttctttgctttgcttaatgaagatcaaaacctggtaattaaatttggctaatataatcattccttttctgacaagacttttttcacctttattcacctgagtaacttacctgtttccaaagacacctaggaaattcagaatgttatatatgcttttccttatttactataatttataggacatgagtggatggattctcttcaatagagaaaatgattttctctaattaaaatgcaccaaattgatgtactaagagattgctttagatgaacacatttatgttcagtgaagattatgtggtcttcaatgacactgcaatataattactaggtacaaaacaaaagcagagatccacacacaatggctcactgtcttcgatgacaacacttttaggatctcatttattcattctttaagtaatttttcttttaaaaaagggataggtggaaaaaatagttgggaaatctttaactaggctaaggtttagacataggtataaattatttattttgtaacattcaaaaaccaaaaaccaccctgacatactgggtggcaagaaaagtcaagatcagattaaacatttgttttgcactaatcacaaaactaataatccaagtcactatcatcaactccagttgatctcagctctgattatgcatcagaacaccctgtgaggtctattaagttcctataccaaatcccaaacactcttgaatcagtctacaaagttgggacctaggtatctgtacattttttaaagttcctcaaaaaattctgcttctaggcaaatgtaatagatattgtgcgttgctcatgtttttcctatcagaaccatgattttaaaaaaactatcctttctgtccccatatatccctcatgtggcctccacttctactctcagctccagtggacctgactgccctaaaggttattctagaccctttgccagtgactggctcagggatggacaggtctaagttactttagagcaatgagacctaaggatatggaaagtgaattctgggaaagctttctcatactaggacagggcccctagaatccagcctgactcttccgctgcatgtaaatgaagatgcacaaggctccaactgctactggcaatcatcccatgaccacgagggtagccagccttaggatgatgccaatgttgtggttgaaaagggggtggggtgtggaggcgggttcccaaggttcttgatgacattactgaatcattggatcagaaacactgcagcacattctgtcaatagatttcatgtattgtgaatcaatatattttcttactgtttttaagtcattttaagttggacttttagtggtcagcatctgaatgttaaagagtggtcccagcacagcattctttaattataacaatctgtatcaagtagaatccacacaaacaccccttcgtacttacataatctgtaaatctgatgtatctttcctattttaacaaaatctttaatttatatcgttataccttactaaagtgttaatgtgcattgcattcacttcattatttactcagagttcttgctgtaggctttgtcttgaatgtgtaggaccattcgtcgtgcatagaagtccctatattcctctggtaactcggccagtgttttcaaggctctgtccagaatttgtgcagctcttgatgctgctgtaggatctttgtttccataggtatctgttttatcatagcattcagatggaaggtgcttccaaaagatattcactcccactccaaactcttcagaaattacattatggaaccataaagcaggaatgaataatacatcaccagcttcaagggaacattcatatcttctagccttggaaaaaagtggatatttagccaagtctgggttatctatattcagtacttctgatttagtaccttttaaatataaatactgggcatctcgaggactgaagagtacaacacgcttttttcctgtcacttgtattaacaaattatccattacatcataatgagtccatagttgtaatcctggtgaactaattcgaaaaacactggaaaagaactgttcctctttgaagaattctggaaacttaatatctcctttcaacaaaggaaactgctttctgatatctgcaacatcctttctagggtcttctccaagtgaccgtaagtagtatttctcatcctctgaaacaaagaattctttatgtttctcttcagctgccctctggaccaactggtcaaaaggtaaagttctgtgggtagaggtgctgcatgaactgctcccgagaaacgccctccagccggggtaccgggaggtgctgcccggccatggttgctcacgcctgccctct

SEQ ID NO: 16034 - RNA, 3449 nt, Homo sapiens
  source 1..3449: mol_type = other RNA
gctgggattacaggcatgagccatggcacctgacccaccattacttttattttgaatcttgtctgtgtagcaagcagtgcagtgagaaattttgttggcagaggaaaaaaattcctttttgcatcaggtcaagcccccaaactagccaaagaaaagctgtgtaatctattcagaagtactggagatgtgctgcacattagggagaatggagaattactggtcacaacgaatcccggtttctatcacccatagctatgtgaacccagacaatcattaagcaatctgggttggttagatggcttctaagatctctttcaataaaaaagttctaagattcagaattcctgagaagttgcagctaacatacactgtataagattttatacattaaaaacaaacatctcatttggtcttaacccagtaggaagaaaagattaaaatattttgtatttgaaataaacagaccctaatattaattatgaccagggaaataattttaaaacatcccaaaggaaagttctctaacttttaaaatattataaattaatactgcaacaggagctacctcaaatctctcaacaaagatggaatataattaaatagaagaactagcaccagttatcaactatgtgcctgcccttgaactctctgcatttttgtagttctgttttaaagatgaggaaaataagcttcatagataaatgttattttgtctaaggtcatccagtttgcttctccattaaacaatcaattaagatgactattcagtgcacaaactgtaatctgttttattaatacttccaagttttctacatgactctggatttatactttgtatcaattctcttgctggttaagaaaaaaaacaagatttattaaaaactgaccataaataatgtgtaaactaaggagagttttgtctttttccttactgaaggacaaggaatcagtaaagaagttctttgctttgcttaatgaagatcaaaacctggtaattaaatttggctaatataatcattccttttctgacaagacttttttcacctttattcacctgagtaacttacctgtttccaaagacacctaggaaattcagaatgttatatatgcttttccttatttactataatttataggacatgagtggatggattctcttcaatagagaaaatgattttctctaattaaaatgcaccaaattgatgtactaagagattgctttagatgaacacatttatgttcagtgaagattatgtggtcttcaatgacactgcaatataattactaggtacaaaacaaaagcagagatccacacacaatggctcactgtcttcgatgacaacacttttaggatctcatttattcattctttaagtaatttttcttttaaaaaagggataggtggaaaaaatagttgggaaatctttaactaggctaaggtttagacataggtataaattatttattttgtaacattcaaaaaccaaaaaccaccctgacatactgggtggcaagaaaagtcaagatcagattaaacatttgttttgcactaatcacaaaactaataatccaagtcactatcatcaactccagttgatctcagctctgattatgcatcagaacaccctgtgaggtctattaagttcctataccaaatcccaaacactcttgaatcagtctacaaagttgggacctaggtatctgtacattttttaaagttcctcaaaaaattctgcttctaggcaaatgtaatagatattgtgcgttgctcatgtttttcctatcagaaccatgattttaaaaaaactatcctttctgtccccatatatccctcatgtggcctccacttctactctcagctccagtggacctgactgccctaaaggttattctagaccctttgccagtgactggctcagggatggacaggtctaagttactttagagcaatgagacctaaggatatggaaagtgaattctgggaaagctttctcatactaggacagggcccctagaatccagcctgactcttccgctgcatgtaaatgaagatgcacaaggctccaactgctactggcaatcatcccatgaccacgagggtagccagccttaggatgatgccaatgttgtggttgaaaagggggtggggtgtggaggcgggttcccaaggttcttgatgacattactgaatcattggatcagaaacactgcagcacattctgtcaatagatttcatgtattgtgaatcaatatattttcttactgtttttaagtcattttaagttggacttttagtggtcagcatctgaatgttaaagagtggtcccagcacagcattctttaattataacaatctgtatcaagtagaatccacacaaacaccccttcgtacttacataatctgtaaatctgatgtatctttcctattttaacaaaatctttaatttatatcgttataccttactaaagtgttaatgtgcattgcattcacttcattatttactcagagttcttgctgtaggctttgtcttgaatgtgtaggaccattcgtcgtgcatagaagtccctatattcctctggtaactcggccagtgttttcaaggctctgtccagaatttgtgcagctcttgatgctgctgtaggatctttgtttccataggtatctgttttatcatagcattcagatggaaggtgcttccaaaagatattcactcccactccaaactcttcagaaattacattatggaaccataaagcaggaatgaataatacatcaccagcttcaagggaacattcatatcttctagccttggaaaaaagtggatatttagccaagtctgggttatctatattcagtacttctgatttagtaccttttaaatataaatactgggcatctcgaggactgaagagtacaacacgcttttttcctgtcacttgtattaacaaattatccattacatcataatgagtccatagttgtaatcctggtgaactaattcgaaaaacactggaaaagaactgttcctctttgaagaattctggaaacttaatatctcctttcaacaaaggaaactgctttctgatatctgcaacatcctttctagggtcttctccaagtgaccgtaagtagtatttctcatcctctgaaacaaagaattctttatgtttctcttcagctgccctctggaccaactggtcaaaaggtaaagtttaatgaagtccatctgtgcaactgcagcaacatgaatctttacttctttcttccctccaacttggcttaggtaatccactgtccatttgcttgtacatggccccaaatcaatcccttccaacacaagaggttttctctgtgggtagaggtgctgcatgaactgctcccgagaaacgccctccagccggggtaccgggaggtgctgcccggccatggttgctcacgcctgccctct

SEQ ID NO: 16035 - RNA, 3460 nt, Homo sapiens
  source 1..3460: mol_type = other RNA
gctgggattacaggcatgagccatggcacctgacccaccattacttttattttgaatcttgtctgtgtagcaagcagtgcagtgagaaattttgttggcagaggaaaaaaattcctttttgcatcaggtcaagcccccaaactagccaaagaaaagctgtgtaatctattcagaagtactggagatgtgctgcacattagggagaatggagaattactggtcacaacgaatcccggtttctatcacccatagctatgtgaacccagacaatcattaagcaatctgggttggttagatggcttctaagatctctttcaataaaaaagttctaagattcagaattcctgagaagttgcagctaacatacactgtataagattttatacattaaaaacaaacatctcatttggtcttaacccagtaggaagaaaagattaaaatattttgtatttgaaataaacagaccctaatattaattatgaccagggaaataattttaaaacatcccaaaggaaagttctctaacttttaaaatattataaattaatactgcaacaggagctacctcaaatctctcaacaaagatggaatataattaaatagaagaactagcaccagttatcaactatgtgcctgcccttgaactctctgcatttttgtagttctgttttaaagatgaggaaaataagcttcatagataaatgttattttgtctaaggtcatccagtttgcttctccattaaacaatcaattaagatgactattcagtgcacaaactgtaatctgttttattaatacttccaagttttctacatgactctggatttatactttgtatcaattctcttgctggttaagaaaaaaaacaagatttattaaaaactgaccataaataatgtgtaaactaaggagagttttgtctttttccttactgaaggacaaggaatcagtaaagaagttctttgctttgcttaatgaagatcaaaacctggtaattaaatttggctaatataatcattccttttctgacaagacttttttcacctttattcacctgagtaacttacctgtttccaaagacacctaggaaattcagaatgttatatatgcttttccttatttactataatttataggacatgagtggatggattctcttcaatagagaaaatgattttctctaattaaaatgcaccaaattgatgtactaagagattgctttagatgaacacatttatgttcagtgaagattatgtggtcttcaatgacactgcaatataattactaggtacaaaacaaaagcagagatccacacacaatggctcactgtcttcgatgacaacacttttaggatctcatttattcattctttaagtaatttttcttttaaaaaagggataggtggaaaaaatagttgggaaatctttaactaggctaaggtttagacataggtataaattatttattttgtaacattcaaaaaccaaaaaccaccctgacatactgggtggcaagaaaagtcaagatcagattaaacatttgttttgcactaatcacaaaactaataatccaagtcactatcatcaactccagttgatctcagctctgattatgcatcagaacaccctgtgaggtctattaagttcctataccaaatcccaaacactcttgaatcagtctacaaagttgggacctaggtatctgtacattttttaaagttcctcaaaaaattctgcttctaggcaaatgtaatagatattgtgcgttgctcatgtttttcctatcagaaccatgattttaaaaaaactatcctttctgtccccatatatccctcatgtggcctccacttctactctcagctccagtggacctgactgccctaaaggttattctagaccctttgccagtgactggctcagggatggacaggtctaagttactttagagcaatgagacctaaggatatggaaagtgaattctgggaaagctttctcatactaggacagggcccctagaatccagcctgactcttccgctgcatgtaaatgaagatgcacaaggctccaactgctactggcaatcatcccatgaccacgagggtagccagccttaggatgatgccaatgttgtggttgaaaagggggtggggtgtggaggcgggttcccaaggttcttgatgacattactgaatcattggatcagaaacactgcagcacattctgtcaatagatttcatgtattgtgaatcaatatattttcttactgtttttaagtcattttaagttggacttttagtggtcagcatctgaatgttaaagagtggtcccagcacagcattctttaattataacaatctgtatcaagtagaatccacacaaacaccccttcgtacttacataatctgtaaatctgatgtatctttcctattttaacaaaatctttaatttatatcgttataccttactaaagtgttaatgtgcattgcattcacttcattatttactcagagttcttgctgtaggctttgtcttgaatgtgtaggaccattcgtcgtgcatagaagtccctatattcctctggtaactcggccagtgttttcaaggctctgtccagaatttgtgcagctcttgatgctgctgtaggatctttgtttccataggtatctgttttatcatagcattcagatggaaggtgcttccaaaagatattcactcccactccaaactcttcagaaattacattatggaaccataaagcaggaatgaataatacatcaccagcttcaagggaacattcatatcttctagccttggaaaaaagtggatatttagccaagtctgggttatctatattcagtacttctgatttagtaccttttaaatataaatactgggcatctcgaggactgaagagtacaacacgcttttttcctgtcacttgtattaacaaattatccattacatcataatgagtccatagttgtaatcctggtgaactaattcgaaaaacactggaaaagaactgttcctctttgaagaattctggaaacttaatatctcctttcaacaaaggaaactgctttctgatatctgcaacatctaatgaagtccatctgtgcaactgcagcaacatgaatctttacttctttcttccctccaacttggcttaggtaatccactgtccatttgcttgtacatggccccaaatcaatcccttccaacacaagaggttttctctgtgggtagaggtgctgcatgaactgctcccgagaaacgccctccagccggggtaccgggaggtgctgcccggccatggttgctcacgcctgccctcttccaggtcttcggaacttcggctctaaagcgttcctcagcgccatccgcccggaaacacgagcgacagagaaaaggtccgcgaggccggcagactccagagtggctgggtccgagcgcggggcggg

SEQ ID NO: 16036 - RNA, 3303 nt, Homo sapiens
  source 1..3303: mol_type = other RNA
gctgggattacaggcatgagccatggcccccagtgcaatcctcttaacataaacagtttaatggcaattaatgcttgaaatcaatgttaaatcaacaaactcaggtcaaggctgatttgactctaatgtcaattaatgcttgatggtttgctatactcactgcatttgaaacaactgtctccaaaaggaattgtctgatggtctgcaaggagtgaccttggactgaagacccttccacactgatgacatttgtaagatttctgtccagcatggattctctgatgtctaatgaggtgtgaatgtgaagtaaacgctttgccacaatcatcacacttgtgaggtttctctcctgtatgaatcctcctatgttttgcataggatgaagcttgactgaagaccttgcctcaatcatgacatttataaggtttctctccagcatgagttcaccagtgaaatgcaaggcatgaacgatgtctgaaaaatttgccacatttattacacttgtaagatctcttcactgtggattctccaatgatgtgcaatggttgtagcattactgaaaactttgtgacaatcattacattagtcaagtttccctataccatggattgcttgatggtgaataagtggtgactgcccactaaagggtttgccacactcattgcacttgtaaggtttctctccagtgtgaattctagtatggggtgccacgtgtgaatcattcccgaaagccttgtcacaaaccttacatttctatggcttttctccagtgtgaattctcctatgtatttgaagctggatttgtgaatgaaaactttgtcacattgttcacgtttgtaagatttctatgcagtatgaagtctatgatgacttgcaaggtgtgattgttgattaaaaaccatgtcacattcattgtgcttgtaaggtttctctccactatgaattacaaggtgtgaattttgaccttttaattacaaggtgtgaattttgaccaacggtcttgccacactcattacacttataatgagtttctctccagtgtgaattctagtatgttttgccagatatgcattatatgcaaaaaccttgtcacaaaccttacctctgtatggtttctcttcaatgtgaattttcttatgtgttttaaggtttgatttacaactgaaaacttttgtcacattcctcccatttgtaaggtttctctccagtatgaagtctatggtgatgtgcaaaggttgctttttgattaaaaaccttgccacattcattatgcttgtaaggtttctctccagtatgaattgccttatgacttacagggttgaattgtgatggaaggtcttgccacactcattacactattaaggcttctctccactatgaagcctatgatggtatacaagggatgacatctgactgaaggtcttgccacactcattacacttgtaaggtttctctccagtatgaagcctacgatggattataagcgatgatgtctgaccgaaggtcttgccacactcattacacttgtaaggtttctctccagtatgaactctctgatgttgtgccaggtgtgaatccctctggaaagccttgtcacaaaccttacatttgtatggtttctctccagtatgaatcctcctgtgtctttccaggtttgatttgcgactgaaaactttgcaacattcttcacatttgtaaggtttctctccactatgaatcctcctatgtctttcaaggtgtgatttgcgactgaaaactttgtcacactcttcacatttgtaaggtttctctccagtatgaagtctatgatggcgtgcaagggttgatagtcgattaaaaactttgccacattcattacatgtgtaaggtttctctccagtgtgaagtatagtatgttttgccagatatgaattatatgcgaaagcctcatcacaaaccttacatttgtatggtttctctccagtatgaatcctcttatgtctttcaaggtgtgatttgcgactgaaaactttgtcacattcttcacattcataaggtttctctccagtatgaagcgctttgtgaatgaagagggatgaattatgaccaaaggtcttgccacactcattacacttgtaaggtttctcaccagtgtgacatctacgatggcaggcaaggtatcgcttctgattaaagaccttgccacatacatcacatttacattgtttctcttctaagtgaattatctgatgtttttttaagagtgagctgcaattaaaggatttgaagctctgtatacattcaaaagatttttctctcatgtgtacttcccatttttgtgtgagtaatgaagaatggagggaattatttccatacttattagaaatatgggttttgggcctacaacaaattctttgggatgttgaaactgaggaagcattgttgatagacttctcaacttgattaccaattttcccttcagactgaaatatgtgcggttcaggcagatgcaaatgaaagcttgatccaagctgatctttaatacgcttgtttccagcatgcctttgatcatgttggcctgtactaccagccaactctttgatttctgtcatgggtgctgcatggccatttgtttcatcttctttccactgaaactcgaagccatgaatgtctttctcaatttcatggaaacaaaattctccaatgtgatgacttgcttgtctgtgcaatgtccctgtgtggatcacttctgtattgccttgccctgttgacgacaacgtcttcaacatgcatttggaagagatatccagggagacgaggttcctataattctccagcatcacgtccctgtataaagtcctctgagcagggtccaggcatttccactcctcctgagagaattctatggccacgtccctgaatgtcaatagacccacgtacttcgtgcatattaatacgtgactcccattggcagctgctccaatcctggtccacagtgagctgacagtgcatccagatgtggcccctgaacaatccctgctgcccaagagcactgacaccacaggaccctcaccccgtgtccatccatgtcggggtgtgagcccttcccaggacctgcccagtgcagcctcttcccaagttcatgacactgggtcacgagagacggaacctaagcgagatgagagggactgaggaagagccatccctgactcctttgctttcctcttcctcttctgggtttctttctcacgtaccaacagtctttagaagtcaatccgcccgccgcggcgtgaccgtcattccacgggatccacttcctggtct

SEQ ID NO: 16037 - RNA, 3048 nt, Homo sapiens
  source 1..3048: mol_type = other RNA
gctgggattacaggcatgagccatggcccccagtgcaatcctcttaacataaacagtttaatggcaattaatgcttgaaatcaatgttaaatcaacaaactcaggtcaaggctgatttgactctaatgtcaattaatgcttgatggtttgctatactcactgcatttgaaacaactgtctccaaaaggaattgtctgatggtctgcaaggagtgaccttggactgaagacccttccacactgatgacatttgtaagatttctgtccagcatggattctctgatgtctaatgaggtgtgaatgtgaagtaaacgctttgccacaatcatcacacttgtgaggtttctctcctgtatgaatcctcctatgttttgcataggatgaagcttgactgaagaccttgcctcaatcatgacatttataaggtttctctccagcatgagttcaccagtgaaatgcaaggcatgaacgatgtctgaaaaatttgccacatttattacacttgtaagatctcttcactgtggattctccaatgatgtgcaatggttgtagcattactgaaaactttgtgacaatcattacattagtcaagtttccctataccatggattgcttgatggtgaataagtggtgactgcccactaaagggtttgccacactcattgcacttgtaaggtttctctccagtgtgaattctagtatggggtgccacgtgtgaatcattcccgaaagccttgtcacaaaccttacatttctatggcttttctccagtgtgaattctcctatgtatttgaagctggatttgtgaatgaaaactttgtcacattgttcacgtttgtaagatttctatgcagtatgaagtctatgatgacttgcaaggtgtgattgttgattaaaaaccatgtcacattcattgtgcttgtaaggtttctctccactatgaattacaaggtgtgaattttgaccttttaattacaaggtgtgaattttgaccaacggtcttgccacactcattacacttataatgagtttctctccagtgtgaattctagtatgttttgccagatatgcattatatgcaaaaaccttgtcacaaaccttacctctgtatggtttctcttcaatgtgaattttcttatgtgttttaaggtttgatttacaactgaaaacttttgtcacattcctcccatttgtaaggtttctctccagtatgaagtctatggtgatgtgcaaaggttgctttttgattaaaaaccttgccacattcattatgcttgtaaggtttctctccagtatgaattgccttatgacttacagggttgaattgtgatggaaggtcttgccacactcattacactattaaggcttctctccactatgaagcctatgatggtatacaagggatgacatctgactgaaggtcttgccacactcattacacttgtaaggtttctctccagtatgaagcctacgatggattataagcgatgatgtctgaccgaaggtcttgccacactcattacacttgtaaggtttctctccagtatgaactctctgatgttgtgccaggtgtgaatccctctggaaagccttgtcacaaaccttacatttgtatggtttctctccagtatgaatcctcctgtgtctttccaggtttgatttgcgactgaaaactttgcaacattcttcacatttgtaaggtttctctccactatgaatcctcctatgtctttcaaggtgtgatttgcgactgaaaactttgtcacactcttcacatttgtaaggtttctctccagtatgaagtctatgatggcgtgcaagggttgatagtcgattaaaaactttgccacattcattacatgtgtaaggtttctctccagtgtgaagtatagtatgttttgccagatatgaattatatgcgaaagcctcatcacaaaccttacatttgtatggtttctctccagtatgaatcctcttatgtctttcaaggtgtgatttgcgactgaaaactttgtcacattcttcacattcataaggtttctctccagtatgaagcgctttgtgaatgaagagggatgaattatgaccaaaggtcttgccacactcattacacttgtaaggtttctcaccagtgtgacatctacgatggcaggcaaggtatcgcttctgattaaagaccttgccacatacatcacatttacattgtttctcttctaagtgaattatctgatgtttttttaagagtgagctgcaattaaaggatttgaagctctgtatacattcaaaagatttttctctcatgtgtacttcccatttttgtgtgagtaatgaagaatggagggaattatttccatacttattagaaatatgggttttgggcctacaacaaattctttgggatgttgaaactgaggaagcattgttgatagacttctcaacttgattaccaattttcccttcagactgaaatatgtgcggttcaggcagatgcaaatgaaagcttgatccaagctgatctttaatacgcttgtttccagcatgcctttgatcatgttggcctgtactaccagccaactctttgatttctgtcatgggtgctgcatggccatttgtttcatcttctttccactgaaactcgaagccatgaatgtctttctcaatttcatggaaacaaaattctccaatgtgatgacttgcttgtctgtgcaatgtccctgtgtggatcacttctgtattgccttgccctgttgacgacaacgtcttcaacatgcatttggaagagatatccagggagacgaggttcctataattctccagcatcacgtccctgtataaagtcctctgagcagggtccaggcatttccactcctcctgagagaattctatggccacgtccctgaatgtcaatagaccctgaggaagagccatccctgactcctttgctttcctcttcctcttctgggtttctttctcacgtaccaacagtctttagaagtcaatccgcccgccgcggcgtgaccgtcattccacgggatccacttcctggtct

SEQ ID NO: 16038 - RNA, 3293 nt, Homo sapiens
  source 1..3293: mol_type = other RNA
gctgggattacaggcatgagccatggcccccagtgcaatcctcttaacataaacagtttaatggcaattaatgcttgaaatcaatgttaaatcaacaaactcaggtcaaggctgatttgactctaatgtcaattaatgcttgatggtttgctatactcactgcatttgaaacaactgtctccaaaaggaattgtctgatggtctgcaaggagtgaccttggactgaagacccttccacactgatgacatttgtaagatttctgtccagcatggattctctgatgtctaatgaggtgtgaatgtgaagtaaacgctttgccacaatcatcacacttgtgaggtttctctcctgtatgaatcctcctatgttttgcataggatgaagcttgactgaagaccttgcctcaatcatgacatttataaggtttctctccagcatgagttcaccagtgaaatgcaaggcatgaacgatgtctgaaaaatttgccacatttattacacttgtaagatctcttcactgtggattctccaatgatgtgcaatggttgtagcattactgaaaactttgtgacaatcattacattagtcaagtttccctataccatggattgcttgatggtgaataagtggtgactgcccactaaagggtttgccacactcattgcacttgtaaggtttctctccagtgtgaattctagtatggggtgccacgtgtgaatcattcccgaaagccttgtcacaaaccttacatttctatggcttttctccagtgtgaattctcctatgtatttgaagctggatttgtgaatgaaaactttgtcacattgttcacgtttgtaagatttctatgcagtatgaagtctatgatgacttgcaaggtgtgattgttgattaaaaaccatgtcacattcattgtgcttgtaaggtttctctccactatgaattacaaggtgtgaattttgaccttttaattacaaggtgtgaattttgaccaacggtcttgccacactcattacacttataatgagtttctctccagtgtgaattctagtatgttttgccagatatgcattatatgcaaaaaccttgtcacaaaccttacctctgtatggtttctcttcaatgtgaattttcttatgtgttttaaggtttgatttacaactgaaaacttttgtcacattcctcccatttgtaaggtttctctccagtatgaagtctatggtgatgtgcaaaggttgctttttgattaaaaaccttgccacattcattatgcttgtaaggtttctctccagtatgaattgccttatgacttacagggttgaattgtgatggaaggtcttgccacactcattacactattaaggcttctctccactatgaagcctatgatggtatacaagggatgacatctgactgaaggtcttgccacactcattacacttgtaaggtttctctccagtatgaagcctacgatggattataagcgatgatgtctgaccgaaggtcttgccacactcattacacttgtaaggtttctctccagtatgaactctctgatgttgtgccaggtgtgaatccctctggaaagccttgtcacaaaccttacatttgtatggtttctctccagtatgaatcctcctgtgtctttccaggtttgatttgcgactgaaaactttgcaacattcttcacatttgtaaggtttctctccactatgaatcctcctatgtctttcaaggtgtgatttgcgactgaaaactttgtcacactcttcacatttgtaaggtttctctccagtatgaagtctatgatggcgtgcaagggttgatagtcgattaaaaactttgccacattcattacatgtgtaaggtttctctccagtgtgaagtatagtatgttttgccagatatgaattatatgcgaaagcctcatcacaaaccttacatttgtatggtttctctccagtatgaatcctcttatgtctttcaaggtgtgatttgcgactgaaaactttgtcacattcttcacattcataaggtttctctccagtatgaagcgctttgtgaatgaagagggatgaattatgaccaaaggtcttgccacactcattacacttgtaaggtttctcaccagtgtgacatctacgatggcaggcaaggtatcgcttctgattaaagaccttgccacatacatcacatttacattgtttctcttctaagtgaattatctgatgtttttttaagagtgagctgcaattaaaggatttgaagctctgtatacattcaaaagatttttctctcatgtgtacttcccatttttgtgtgagtaatgaagaatggagggaattatttccatacttattagaaatatgggttttgggcctacaacaaattctttgggatgttgaaactgaggaagcattgttgatagacttctcaacttgattaccaattttcccttcagactgaaatatgtgcggttcaggcagatgcaaatgaaagcttgatccaagctgatctttaatacgcttgtttccagcatgcctttgatcatgttggcctgtactaccagccaactctttgatttctgtcatgggtgctgcatggccatttgtttcatcttctttccactgaaactcgaagccatgaatgtctttctcaatttcatggaaacaaaattctccaatgtgatgacttgcttgtctgtgcaatgtccctgtgtggatcacttctgtattgccttgccctgttgacgacaacgtcttcaacatgcatttggaagagatatccagggagacgaggttcctataattctccagcatcacgtccctgtataaagtcctctgagcagggtccaggcatttccactcctcctgagagaattctatggccacgtccctgaatgtcaatagaccttcgtgcatattaatacgtgactcccattggcagctgctccaatcctggtccacagtgagctgacagtgcatccagatgtggcccctgaacaatccctgctgcccaagagcactgacaccacaggaccctcaccccgtgtccatccatgtcggggtgtgagcccttcccaggacctgcccagtgcagcctcttcccaagttcatgacactgggtcacgagagacggaacctaagcgagatgagagggactgaggaagagccatccctgactcctttgctttcctcttcctcttctgggtttctttctcacgtaccaacagtctttagaagtcaatccgcccgccgcggcgtgaccgtcattccacgggatccacttcctgg

SEQ ID NO: 16039 - RNA, 3421 nt, Homo sapiens
  source 1..3421: mol_type = other RNA
gctgggattacaggcatgagccatggcccccagtgcaatcctcttaacataaacagtttaatggcaattaatgcttgaaatcaatgttaaatcaacaaactcaggtcaaggctgatttgactctaatgtcaattaatgcttgatggtttgctatactcactgcatttgaaacaactgtctccaaaaggaattgtctgatggtctgcaaggagtgaccttggactgaagacccttccacactgatgacatttgtaagatttctgtccagcatggattctctgatgtctaatgaggtgtgaatgtgaagtaaacgctttgccacaatcatcacacttgtgaggtttctctcctgtatgaatcctcctatgttttgcataggatgaagcttgactgaagaccttgcctcaatcatgacatttataaggtttctctccagcatgagttcaccagtgaaatgcaaggcatgaacgatgtctgaaaaatttgccacatttattacacttgtaagatctcttcactgtggattctccaatgatgtgcaatggttgtagcattactgaaaactttgtgacaatcattacattagtcaagtttccctataccatggattgcttgatggtgaataagtggtgactgcccactaaagggtttgccacactcattgcacttgtaaggtttctctccagtgtgaattctagtatggggtgccacgtgtgaatcattcccgaaagccttgtcacaaaccttacatttctatggcttttctccagtgtgaattctcctatgtatttgaagctggatttgtgaatgaaaactttgtcacattgttcacgtttgtaagatttctatgcagtatgaagtctatgatgacttgcaaggtgtgattgttgattaaaaaccatgtcacattcattgtgcttgtaaggtttctctccactatgaattacaaggtgtgaattttgaccttttaattacaaggtgtgaattttgaccaacggtcttgccacactcattacacttataatgagtttctctccagtgtgaattctagtatgttttgccagatatgcattatatgcaaaaaccttgtcacaaaccttacctctgtatggtttctcttcaatgtgaattttcttatgtgttttaaggtttgatttacaactgaaaacttttgtcacattcctcccatttgtaaggtttctctccagtatgaagtctatggtgatgtgcaaaggttgctttttgattaaaaaccttgccacattcattatgcttgtaaggtttctctccagtatgaattgccttatgacttacagggttgaattgtgatggaaggtcttgccacactcattacactattaaggcttctctccactatgaagcctatgatggtatacaagggatgacatctgactgaaggtcttgccacactcattacacttgtaaggtttctctccagtatgaagcctacgatggattataagcgatgatgtctgaccgaaggtcttgccacactcattacacttgtaaggtttctctccagtatgaactctctgatgttgtgccaggtgtgaatccctctggaaagccttgtcacaaaccttacatttgtatggtttctctccagtatgaatcctcctgtgtctttccaggtttgatttgcgactgaaaactttgcaacattcttcacatttgtaaggtttctctccactatgaatcctcctatgtctttcaaggtgtgatttgcgactgaaaactttgtcacactcttcacatttgtaaggtttctctccagtatgaagtctatgatggcgtgcaagggttgatagtcgattaaaaactttgccacattcattacatgtgtaaggtttctctccagtgtgaagtatagtatgttttgccagatatgaattatatgcgaaagcctcatcacaaaccttacatttgtatggtttctctccagtatgaatcctcttatgtctttcaaggtgtgatttgcgactgaaaactttgtcacattcttcacattcataaggtttctctccagtatgaagcgctttgtgaatgaagagggatgaattatgaccaaaggtcttgccacactcattacacttgtaaggtttctcaccagtgtgacatctacgatggcaggcaaggtatcgcttctgattaaagaccttgccacatacatcacatttacattgtttctcttctaagtgaattatctgatgtttttttaagagtgagctgcaattaaaggatttgaagctctgtatacattcaaaagatttttctctcatgtgtacttcccatttttgtgtgagtaatgaagaatggagggaattatttccatacttattagaaatatgggttttgggcctacaacaaattctttgggatgttgaaactgaggaagcattgttgatagacttctcaacttgattaccaattttcccttcagactgaaatatgtgcggttcaggcagatgcaaatgaaagcttgatccaagctgatctttaatacgcttgtttccagcatgcctttgatcatgttggcctgtactaccagccaactctttgatttctgtcatgggtgctgcatggccatttgtttcatcttctttccactgaaactcgaagccatgaatgtctttctcaatttcatggaaacaaaattctccaatgtgatgacttgcttgtctgtgcaatgtccctgtgtggatcacttctgtattgccttgccctgttgacgacaacgtcttcaacatgcatttggaagagatatctgtagtcccaggtacttggaaggctgaggcaggagaattgcttgaacctgggaagtggaggttgcagtgagcggagatgacaccactgtactttagccgggatgacagaccaaaactccagggagacgaggttcctataattctccagcatcacgtccctgtataaagtcctctgagcagggtccaggcatttccactcctcctgagagaattctatggccacgtccctgaatgtcaatagacccacgtacttcgtgcatattaatacgtgactcccattggcagctgctccaatcctggtccacagtgagctgacagtgcatccagatgtggcccctgaacaatccctgctgcccaagagcactgacaccacaggaccctcaccccgtgtccatccatgtcggggtgtgagcccttcccaggacctgcccagtgcagcctcttcccaagttcatgacactgggtcacgagagacggaacctaagcgagatgagagggactgaggaagagccatccctgactcctttgctttcctcttcctcttctgggtttctttctcacgtaccaacagtctttagaagtcaatccgcccgccgcggcgtgaccgtcattccacgggatccacttcctggtct

SEQ ID NO: 16040 - RNA, 3402 nt, Homo sapiens
  source 1..3402: mol_type = other RNA
gctgggattacaggcatgagccatggcccccagtgcaatcctcttaacataaacagtttaatggcaattaatgcttgaaatcaatgttaaatcaacaaactcaggtcaaggctgatttgactctaatgtcaattaatgcttgatggtttgctatactcactgcatttgaaacaactgtctccaaaaggaattgtctgatggtctgcaaggagtgaccttggactgaagacccttccacactgatgacatttgtaagatttctgtccagcatggattctctgatgtctaatgaggtgtgaatgtgaagtaaacgctttgccacaatcatcacacttgtgaggtttctctcctgtatgaatcctcctatgttttgcataggatgaagcttgactgaagaccttgcctcaatcatgacatttataaggtttctctccagcatgagttcaccagtgaaatgcaaggcatgaacgatgtctgaaaaatttgccacatttattacacttgtaagatctcttcactgtggattctccaatgatgtgcaatggttgtagcattactgaaaactttgtgacaatcattacattagtcaagtttccctataccatggattgcttgatggtgaataagtggtgactgcccactaaagggtttgccacactcattgcacttgtaaggtttctctccagtgtgaattctagtatggggtgccacgtgtgaatcattcccgaaagccttgtcacaaaccttacatttctatggcttttctccagtgtgaattctcctatgtatttgaagctggatttgtgaatgaaaactttgtcacattgttcacgtttgtaagatttctatgcagtatgaagtctatgatgacttgcaaggtgtgattgttgattaaaaaccatgtcacattcattgtgcttgtaaggtttctctccactatgaattacaaggtgtgaattttgaccttttaattacaaggtgtgaattttgaccaacggtcttgccacactcattacacttataatgagtttctctccagtgtgaattctagtatgttttgccagatatgcattatatgcaaaaaccttgtcacaaaccttacctctgtatggtttctcttcaatgtgaattttcttatgtgttttaaggtttgatttacaactgaaaacttttgtcacattcctcccatttgtaaggtttctctccagtatgaagtctatggtgatgtgcaaaggttgctttttgattaaaaaccttgccacattcattatgcttgtaaggtttctctccagtatgaattgccttatgacttacagggttgaattgtgatggaaggtcttgccacactcattacactattaaggcttctctccactatgaagcctatgatggtatacaagggatgacatctgactgaaggtcttgccacactcattacacttgtaaggtttctctccagtatgaagcctacgatggattataagcgatgatgtctgaccgaaggtcttgccacactcattacacttgtaaggtttctctccagtatgaactctctgatgttgtgccaggtgtgaatccctctggaaagccttgtcacaaaccttacatttgtatggtttctctccagtatgaatcctcctgtgtctttccaggtttgatttgcgactgaaaactttgcaacattcttcacatttgtaaggtttctctccactatgaatcctcctatgtctttcaaggtgtgatttgcgactgaaaactttgtcacactcttcacatttgtaaggtttctctccagtatgaagtctatgatggcgtgcaagggttgatagtcgattaaaaactttgccacattcattacatgtgtaaggtttctctccagtgtgaagtatagtatgttttgccagatatgaattatatgcgaaagcctcatcacaaaccttacatttgtatggtttctctccagtatgaatcctcttatgtctttcaaggtgtgatttgcgactgaaaactttgtcacattcttcacattcataaggtttctctccagtatgaagcgctttgtgaatgaagagggatgaattatgaccaaaggtcttgccacactcattacacttgtaaggtttctcaccagtgtgacatctacgatggcaggcaaggtatcgcttctgattaaagaccttgccacatacatcacatttacattgtttctcttctaagtgaattatctgatgtttttttaagagtgagctgcaattaaaggatttgaagctctgtatacattcaaaagatttttctctcatgtgtacttcccatttttgtgtgagtaatgaagaatggagggaattatttccatacttattagaaatatgggttttgggcctacaacaaattctttgggatgttgaaactgaggaagcattgttgatagacttctcaacttgattaccaattttcccttcagactgaaatatgtgcggttcaggcagatgcaaatgaaagcttgatccaagctgatctttaatacgcttgtttccagcatgcctttgatcatgttggcctgtactaccagccaactctttgatttctgtcatgggtgctgcatggccatttgtttcatcttctttccactgaaactcgaagccatgaatgtctttctcaatttcatggaaacaaaattctccaatgtgatgacttgcttgtctgtgcaatgtccctgtgtggatcacttctgtattgccttgccctgttgacgacaacgtcttcaacatgcatttggaagagatatctgtagtcccaggtacttggaaggctgaggcaggagaattgcttgaacctgggaagtggaggttgcagtgagcggagatgacaccactgtactttagccgggatgacagaccaaaactccagggagacgaggttcctataattctccagcatcacgtccctgtataaagtcctctgagcagggtccaggcatttccactcctcctgagagaattctatggccacgtccctgaatgtcaatagacccacgtacttcgtgcatattaatacgtgactcccattggcagctgctccaatcctggtccacagtgagctgacagtgcatccagatgtggcccctgaacaatccctgctgcccaagagcactgacaccacaggaccctcaccccgtgtccatccatgtcggggtgtgagcccttcccaggacctgcccagtgcagcctcttcccaagttcatgacactgggtcacgagagacggaacctgaggaagagccatccctgactcctttgctttcctcttcctcttctgggtttctttctcacgtaccaacagtctttagaagtcaatccgcccgccgcggcgtgaccgtcattccacgggatccacttcctggtct

SEQ ID NO: 16041 - RNA, 3166 nt, Homo sapiens
  source 1..3166: mol_type = other RNA
gctgggattacaggcatgagccatggcccccagtgcaatcctcttaacataaacagtttaatggcaattaatgcttgaaatcaatgttaaatcaacaaactcaggtcaaggctgatttgactctaatgtcaattaatgcttgatggtttgctatactcactgcatttgaaacaactgtctccaaaaggaattgtctgatggtctgcaaggagtgaccttggactgaagacccttccacactgatgacatttgtaagatttctgtccagcatggattctctgatgtctaatgaggtgtgaatgtgaagtaaacgctttgccacaatcatcacacttgtgaggtttctctcctgtatgaatcctcctatgttttgcataggatgaagcttgactgaagaccttgcctcaatcatgacatttataaggtttctctccagcatgagttcaccagtgaaatgcaaggcatgaacgatgtctgaaaaatttgccacatttattacacttgtaagatctcttcactgtggattctccaatgatgtgcaatggttgtagcattactgaaaactttgtgacaatcattacattagtcaagtttccctataccatggattgcttgatggtgaataagtggtgactgcccactaaagggtttgccacactcattgcacttgtaaggtttctctccagtgtgaattctagtatggggtgccacgtgtgaatcattcccgaaagccttgtcacaaaccttacatttctatggcttttctccagtgtgaattctcctatgtatttgaagctggatttgtgaatgaaaactttgtcacattgttcacgtttgtaagatttctatgcagtatgaagtctatgatgacttgcaaggtgtgattgttgattaaaaaccatgtcacattcattgtgcttgtaaggtttctctccactatgaattacaaggtgtgaattttgaccttttaattacaaggtgtgaattttgaccaacggtcttgccacactcattacacttataatgagtttctctccagtgtgaattctagtatgttttgccagatatgcattatatgcaaaaaccttgtcacaaaccttacctctgtatggtttctcttcaatgtgaattttcttatgtgttttaaggtttgatttacaactgaaaacttttgtcacattcctcccatttgtaaggtttctctccagtatgaagtctatggtgatgtgcaaaggttgctttttgattaaaaaccttgccacattcattatgcttgtaaggtttctctccagtatgaattgccttatgacttacagggttgaattgtgatggaaggtcttgccacactcattacactattaaggcttctctccactatgaagcctatgatggtatacaagggatgacatctgactgaaggtcttgccacactcattacacttgtaaggtttctctccagtatgaagcctacgatggattataagcgatgatgtctgaccgaaggtcttgccacactcattacacttgtaaggtttctctccagtatgaactctctgatgttgtgccaggtgtgaatccctctggaaagccttgtcacaaaccttacatttgtatggtttctctccagtatgaatcctcctgtgtctttccaggtttgatttgcgactgaaaactttgcaacattcttcacatttgtaaggtttctctccactatgaatcctcctatgtctttcaaggtgtgatttgcgactgaaaactttgtcacactcttcacatttgtaaggtttctctccagtatgaagtctatgatggcgtgcaagggttgatagtcgattaaaaactttgccacattcattacatgtgtaaggtttctctccagtgtgaagtatagtatgttttgccagatatgaattatatgcgaaagcctcatcacaaaccttacatttgtatggtttctctccagtatgaatcctcttatgtctttcaaggtgtgatttgcgactgaaaactttgtcacattcttcacattcataaggtttctctccagtatgaagcgctttgtgaatgaagagggatgaattatgaccaaaggtcttgccacactcattacacttgtaaggtttctcaccagtgtgacatctacgatggcaggcaaggtatcgcttctgattaaagaccttgccacatacatcacatttacattgtttctcttctaagtgaattatctgatgtttttttaagagtgagctgcaattaaaggatttgaagctctgtatacattcaaaagatttttctctcatgtgtacttcccatttttgtgtgagtaatgaagaatggagggaattatttccatacttattagaaatatgggttttgggcctacaacaaattctttgggatgttgaaactgaggaagcattgttgatagacttctcaacttgattaccaattttcccttcagactgaaatatgtgcggttcaggcagatgcaaatgaaagcttgatccaagctgatctttaatacgcttgtttccagcatgcctttgatcatgttggcctgtactaccagccaactctttgatttctgtcatgggtgctgcatggccatttgtttcatcttctttccactgaaactcgaagccatgaatgtctttctcaatttcatggaaacaaaattctccaatgtgatgacttgcttgtctgtgcaatgtccctgtgtggatcacttctgtattgccttgccctgttgacgacaacgtcttcaacatgcatttggaagagatatctgtagtcccaggtacttggaaggctgaggcaggagaattgcttgaacctgggaagtggaggttgcagtgagcggagatgacaccactgtactttagccgggatgacagaccaaaactccagggagacgaggttcctataattctccagcatcacgtccctgtataaagtcctctgagcagggtccaggcatttccactcctcctgagagaattctatggccacgtccctgaatgtcaatagaccctgaggaagagccatccctgactcctttgctttcctcttcctcttctgggtttctttctcacgtaccaacagtctttagaagtcaatccgcccgccgcggcgtgaccgtcattccacgggatccacttcctggtct

SEQ ID NO: 16042 - RNA, 3411 nt, Homo sapiens
  source 1..3411: mol_type = other RNA
gctgggattacaggcatgagccatggcccccagtgcaatcctcttaacataaacagtttaatggcaattaatgcttgaaatcaatgttaaatcaacaaactcaggtcaaggctgatttgactctaatgtcaattaatgcttgatggtttgctatactcactgcatttgaaacaactgtctccaaaaggaattgtctgatggtctgcaaggagtgaccttggactgaagacccttccacactgatgacatttgtaagatttctgtccagcatggattctctgatgtctaatgaggtgtgaatgtgaagtaaacgctttgccacaatcatcacacttgtgaggtttctctcctgtatgaatcctcctatgttttgcataggatgaagcttgactgaagaccttgcctcaatcatgacatttataaggtttctctccagcatgagttcaccagtgaaatgcaaggcatgaacgatgtctgaaaaatttgccacatttattacacttgtaagatctcttcactgtggattctccaatgatgtgcaatggttgtagcattactgaaaactttgtgacaatcattacattagtcaagtttccctataccatggattgcttgatggtgaataagtggtgactgcccactaaagggtttgccacactcattgcacttgtaaggtttctctccagtgtgaattctagtatggggtgccacgtgtgaatcattcccgaaagccttgtcacaaaccttacatttctatggcttttctccagtgtgaattctcctatgtatttgaagctggatttgtgaatgaaaactttgtcacattgttcacgtttgtaagatttctatgcagtatgaagtctatgatgacttgcaaggtgtgattgttgattaaaaaccatgtcacattcattgtgcttgtaaggtttctctccactatgaattacaaggtgtgaattttgaccttttaattacaaggtgtgaattttgaccaacggtcttgccacactcattacacttataatgagtttctctccagtgtgaattctagtatgttttgccagatatgcattatatgcaaaaaccttgtcacaaaccttacctctgtatggtttctcttcaatgtgaattttcttatgtgttttaaggtttgatttacaactgaaaacttttgtcacattcctcccatttgtaaggtttctctccagtatgaagtctatggtgatgtgcaaaggttgctttttgattaaaaaccttgccacattcattatgcttgtaaggtttctctccagtatgaattgccttatgacttacagggttgaattgtgatggaaggtcttgccacactcattacactattaaggcttctctccactatgaagcctatgatggtatacaagggatgacatctgactgaaggtcttgccacactcattacacttgtaaggtttctctccagtatgaagcctacgatggattataagcgatgatgtctgaccgaaggtcttgccacactcattacacttgtaaggtttctctccagtatgaactctctgatgttgtgccaggtgtgaatccctctggaaagccttgtcacaaaccttacatttgtatggtttctctccagtatgaatcctcctgtgtctttccaggtttgatttgcgactgaaaactttgcaacattcttcacatttgtaaggtttctctccactatgaatcctcctatgtctttcaaggtgtgatttgcgactgaaaactttgtcacactcttcacatttgtaaggtttctctccagtatgaagtctatgatggcgtgcaagggttgatagtcgattaaaaactttgccacattcattacatgtgtaaggtttctctccagtgtgaagtatagtatgttttgccagatatgaattatatgcgaaagcctcatcacaaaccttacatttgtatggtttctctccagtatgaatcctcttatgtctttcaaggtgtgatttgcgactgaaaactttgtcacattcttcacattcataaggtttctctccagtatgaagcgctttgtgaatgaagagggatgaattatgaccaaaggtcttgccacactcattacacttgtaaggtttctcaccagtgtgacatctacgatggcaggcaaggtatcgcttctgattaaagaccttgccacatacatcacatttacattgtttctcttctaagtgaattatctgatgtttttttaagagtgagctgcaattaaaggatttgaagctctgtatacattcaaaagatttttctctcatgtgtacttcccatttttgtgtgagtaatgaagaatggagggaattatttccatacttattagaaatatgggttttgggcctacaacaaattctttgggatgttgaaactgaggaagcattgttgatagacttctcaacttgattaccaattttcccttcagactgaaatatgtgcggttcaggcagatgcaaatgaaagcttgatccaagctgatctttaatacgcttgtttccagcatgcctttgatcatgttggcctgtactaccagccaactctttgatttctgtcatgggtgctgcatggccatttgtttcatcttctttccactgaaactcgaagccatgaatgtctttctcaatttcatggaaacaaaattctccaatgtgatgacttgcttgtctgtgcaatgtccctgtgtggatcacttctgtattgccttgccctgttgacgacaacgtcttcaacatgcatttggaagagatatctgtagtcccaggtacttggaaggctgaggcaggagaattgcttgaacctgggaagtggaggttgcagtgagcggagatgacaccactgtactttagccgggatgacagaccaaaactccagggagacgaggttcctataattctccagcatcacgtccctgtataaagtcctctgagcagggtccaggcatttccactcctcctgagagaattctatggccacgtccctgaatgtcaatagaccttcgtgcatattaatacgtgactcccattggcagctgctccaatcctggtccacagtgagctgacagtgcatccagatgtggcccctgaacaatccctgctgcccaagagcactgacaccacaggaccctcaccccgtgtccatccatgtcggggtgtgagcccttcccaggacctgcccagtgcagcctcttcccaagttcatgacactgggtcacgagagacggaacctaagcgagatgagagggactgaggaagagccatccctgactcctttgctttcctcttcctcttctgggtttctttctcacgtaccaacagtctttagaagtcaatccgcccgccgcggcgtgaccgtcattccacgggatccacttcctgg

SEQ ID NO: 16043 - RNA, 838 nt, Homo sapiens
  source 1..838: mol_type = other RNA
gctgggattacaggcatgagccatggcgccccgccatgaaattattttttaactactgtgataatcaactttgatcctaacaatttaagaaatttgtataggaggataagaagaaccctaatctatagggaatgctcatgtccctgaaggaggacaggtcagtaagggcccaaattctctcctggtctttaggtggaaaggcaaaacatcacactttaaaaagaggctgctctcagccaaagcaagaaagacctctttcattaagcctattgatctgaagctattccaggaaggacaaaaaaagttcaagccagatgttcagcagcagccagagttggaccctatgtcacgagagttccgctgggaggcactgggtcccactgatgttgaaattgactgttggggcccaatcttgatgccatttgcctcattgtggacatcaaataaaccctgctggatcttcctatatatttctttggctgtgttaatgaaggcctcttcaacattgcaggctgttttggctgaagtttccatgaatataagtccatgctccctagcaaaggcctctccttcttctctcttcacatccctgcgggactctaggtcactcttattcccaatgagcatgataaccatgttggaactagagtgctgccgggcatcctctaaccatgaggtcaggtggttgaaggtttcacgccttgtaatgtcgtacaccagcagtgctccagctgctccccatattaatctttctgttcccatttctttatcgtatcccagatttgcagtttgatttgttttccatcaatgttgaccatacgagctccaaactccacac

SEQ ID NO: 16044 - RNA, 1012 nt, Homo sapiens
  source 1..1012: mol_type = other RNA
gctgggattacaggcatgagccatggcgccccgccatgaaattattttttaactactgtgataatcaactttgatcctaacaatttaagaaatttgtataggaggataagaagaaccctaatctatagggaatgctcatgtccctgaaggaggacaggtcagtaagggcccaaattctctcctggtctttaggtggaaaggcaaaacatcacactttaaaaagaggctgctctcagccaaagcaagaaagacctctttcattaagcctattgatctgaagctattccaggaaggacaaaaaaagttcaagccagatgttcagcagcagccagagttggaccctatgtcacgagagttccgctgggaggcactgggtcccactgatgttgaaattgactgttggggcccaatcttgatgccatttgcctcattgtggacatcaaataaaccctgctggatcttcctatatatttctttggctgtgttaatgaaggcctcttcaacattgcaggctgttttggctgaagtttccatgaatataagtccatgctccctagcaaaggcctctccttcttctctcttcacatccctgcgggactctaggtcactcttattcccaatgagcatgataaccatgttggaactagagtgctgccgggcatcctctaaccatgaggtcaggtggttgaaggtttcacgccttgtaatgtcgtacaccagcagtgctccagctgctccccgtatcccagatttgcagtttgatttgttttccatcaatgttgaccatacgagctccaaactccacacctattgtgaggtcgtggacaggctggaaccgcttatctgtaaactgcaggaggagacatgacttccccacacctgtgtctccgatgatgatatacttgaagagataagcataagtcatggtgtcgcgtcctctgggttccgggtccgcccgacttctatagccacttacctccgacctctctagccactcaatctaccgatcttc

SEQ ID NO: 16045 - RNA, 998 nt, Homo sapiens
  source 1..998: mol_type = other RNA
gctgggattacaggcatgagccatggcgccccgccatgaaattattttttaactactgtgataatcaactttgatcctaacaatttaagaaatttgtataggaggataagaagaaccctaatctatagggaatgctcatgtccctgaaggaggacaggtcagtaagggcccaaattctctcctggtctttaggtggaaaggcaaaacatcacactttaaaaagaggctgctctcagccaaagcaagaaagacctctttcattaagcctattgatctgaagctattccaggaaggacaaaaaaagttcaagccagatgttcagcagcagccagagttggaccctatgtcacgagagttccgctgggaggcactgggtcccactgatgttgaaattgactgttggggcccaatcttgatgccatttgcctcattgtggacatcaaataaaccctgctggatcttcctatatatttctttggctgtgttaatgaaggcctcttcaacattgcaggctgttttggctgaagtttccatgaatataagtccatgctccctagcaaaggcctctccttcttctctcttcacatccctgcgggactctaggtcactcttattcccaatgagcatgataaccatgttggaactagagtgctgccgggcatcctctaaccatgaggtcaggtggttgaaggtttcacgccttgtaatgtcgtacaccagcagtgctccagctgctcccctgtagtaggaacgggtgatagaacggaaggattcttgcccagccgtatcccagatttgcagtttgatttgttttccatcaatgttgaccatacgagctccaaactccacacctattgtgaggtcgtggacaggctggaaccgcttatctgtaaactgcaggaggagacatgacttccccacacctgaaagagaaagcacactcccggaatcacgcagccctggaacaccttccagagtatggacttcccggaccagag

SEQ ID NO: 16046 - RNA, 1056 nt, Homo sapiens
  source 1..1056: mol_type = other RNA
gctgggattacaggcatgagccatggcgccccgccatgaaattattttttaactactgtgataatcaactttgatcctaacaatttaagaaatttgtataggaggataagaagaaccctaatctatagggaatgctcatgtccctgaaggaggacaggtcagtaagggcccaaattctctcctggtctttaggtggaaaggcaaaacatcacactttaaaaagaggctgctctcagccaaagcaagaaagacctctttcattaagcctattgatctgaagctattccaggaaggacaaaaaaagttcaagccagatgttcagcagcagccagagttggaccctatgtcacgagagttccgctgggaggcactgggtcccactgatgttgaaattgactgttggggcccaatcttgatgccatttgcctcattgtggacatcaaataaaccctgctggatcttcctatatatttctttggctgtgttaatgaaggcctcttcaacattgcaggctgttttggctgaagtttccatgaatataagtccatgctccctagcaaaggcctctccttcttctctcttcacatccctgcgggactctaggtcactcttattcccaatgagcatgataaccatgttggaactagagtgctgccgggcatcctctaaccatgaggtcaggtggttgaaggtttcacgccttgtaatgtcgtacaccagcagtgctccagctgctcccctgtagtaggaacgggtgatagaacggaaggattcttgcccagccgtatcccagatttgcagtttgatttgttttccatcaatgttgaccatacgagctccaaactccacacctattgtgaggtcgtggacaggctggaaccgcttatctgtaaactgcaggaggagacatgacttccccacacctgtgtctccgatgatgatatacttgaagagataagcataagtcatggtgtcgcgtcctctgggttccgggtccgcccgacttctatagccacttacctccgacctctctagccactcaatctaccgatcttc

SEQ ID NO: 16047 - RNA, 1098 nt, Homo sapiens
  source 1..1098: mol_type = other RNA
gctgggattacaggcatgagccatggcgccccgccatgaaattattttttaactactgtgataatcaactttgatcctaacaatttaagaaatttgtataggaggataagaagaaccctaatctatagggaatgctcatgtccctgaaggaggacaggtcagtaagggcccaaattctctcctggtctttaggtggaaaggcaaaacatcacactttaaaaagaggctgctctcagccaaagcaagaaagacctctttcattaagcctattgatctgaagctattccaggaaggacaaaaaaagttcaagccagatgttcagcagcagccagagttggaccctatgtcacgagagttccgctgggaggcactgggtcccactgatgttgaaattgactgttggggcccaatcttgatgccatttgcctcattgtggacatcaaataaaccctgctggatcttcctatatatttctttggctgtgttaatgaaggcctcttcaacattgcaggctgttttggctgaagtttccatgaatataagtccatgctccctagcaaaggcctctccttcttctctcttcacatccctgcgggactctaggtcactcttattcccaatgagcatgataaccatgttggaactagagtgctgccgggcatcctctaaccatgaggtcaggtggttgaaggtttcacgccttgtaatgtcgtacaccagcagtgctccagctgctcccctgtagtaggaacgggtgatagaacggaaggattcttgcccagcctgtggcaccccagtcagcacgataaagacgatgaagacatttgcatacatttcccaatatcctcataaaagaacaactggaaataggactggaaacggagtgtatgtcatttttttcaatcccaaatatgatattgaacacaccatattaatctttctgttcccatttctttatcgtatcccagatttgcagtttgatttgttttccatcaatgttgaccatacgagctccaaactccacacctattgtgaggtcgtggacaggctggaaccgcttatctgtaaactgcaggaggagacatgacttccccacac

SEQ ID NO: 16048 - RNA, 4548 nt, Homo sapiens
  source 1..4548: mol_type = other RNA
gctgggattacaggcatgagccatggcgcctggccccactgtacattttcaatactgctcattgacaacttatctttttctttaagtagggagaatgaacattaagaaacagtatttgtgccgggcatggtggctcacgcctgtaatcccagtgctttgggaggccgaggcaggtggatcacgaggtcaggagattgagaccatactggctaacacagtgaaaccccatttctactaaaaatatgaaaaattagccgggcatggtgatgggcacctgtagtcccagctactcgggaggctgaggcaggaggatggcgtgaatctgggaggcagagcttgcagtgagccacaatcgcgccactgcattctagcctggacaacagagcaagactccgtctcaaaaaaaaaaaaaaaaaaaaaaagaaacagtatttgctatattaggacacaaagagaaaacaaccaaaatcacaaagtccatgtactctggcaaaatactattaaattagaaaaaaatatatcaaatattgtctgatttttttttttttgagacagagttgcactcttttgcccaggctggagtgaagtggcatgatcttggctcactgcaacctccatttcccgggttcaagtgattctccttcctcagcctcttgagtagctgggattatagatgcctgccaccacacccggctaatttttgtattttttagtagaagcggggtttcaccatgttggccaggctggtctcaagctccttacctccggtgatctgcccgcctcagcctcccaaaatgctaggtttataggtgtgagccaccacacctggcaaatgtctaatttctattataacaaactagatcactcaggagctgtttggaaatacctttctgaatatttggtgtattgatgttttagaattataataaatacactgtatataaaacgaggtagtaagattttcaggaccactatagccataaatgtttatattaaaagactgaaaatgaacgagctagtggcccaacctacaaatgagacattgatgaaggtaattccacattcatagcacttacaccttttgttctaagttactgcgtggccactcagttaagagatgaggcatcctaacattgattacgttcctagggcttcctctaaatgaattctctcatgcataaagggaggaatcactgaaaatttttctgaaattaatacactcgtgagtattgcatccaaggaacatttacatatttttcctaatataagaggtatcactgaaaacattccctcatcctttatcttaagaagttctggctgagagtggtagctcgttcctgtattcccagcattttgggaggctgaggcaggtggatcacttgagcccaggagtttgagagcagcctgggaaacatggtgaatccccatctttacaaaaactagacaggcatggtggtgcatgcctacagtcccagctacttgggaggctgaggtgggaggatcccttaagcctgggaggcagaggttacaataagccaagattgcaccactgcactacagcctgggcacagatgaaaccctgtctcaaaaaataaattgtataaattgttatcttacactgagttaggttcctaaaaatgtggaaaaatgacattctaatactgatggaattcaatggtttttctagtatgaatctcacttcttaaaaatggagagaatattcaaggcttttatagcataccaaactatactgtcttgtgcttggtaatatgactgtttgtgtcacaggcttttcaacactgtgtatactcaacatattcctctgttgtatgatctccgaaatgtgacttaaggaatgagtgtcccctggttttccatttttgatgccacacacagggtttccccttattgtgagttgtcatgtgactccctgaagccatcactgaaggctttcctacagctactgcattacctgggcagctccccagtagatactttttttttggtagggggaaagtttgagctcaaagttttaccatacagattacactcacaagatttctctctagagtgagttaacctgtgggtgattgaatgctactcccatattgatcagtttagaagttggctgggcatggtggttcatgcctgtaatcccagtacttctggaggccaagatgaaaggactgcttgaacctaggagtttgagactagtctgggcaacatggcaaaaccctccctctagtttaaaaaaaaacaaattagccagacatggtgtcatgcacctgtagtcccagctacattggaggctggggcaggagaattacttgatcccaggaagtagaggctgcagtgagctgtgatcacaccactgcgctccagactgggtgacagagtgagacattgtcttaaaaaaaaaaaaatgagggtcagctgaaggctttcctccactgatttcatggcaagttttccagatggttccaaatgtctactgttcatacctcctgtggtgttcttccacattgtatcaggattggtgtgtatgaccaatgtaacagggacatgaaaacatatctcactgaagctaggtcataaaagacattatgctttctgtgttggctcctttagatcactggctttggggagaagttgcttccataaagaaactcagccctgttgagaggcctacgtgatttggaagcgcagctcccttggaaacagctagcatgcacttgtcgggcttgtaagccatttggaagtggtcccttcaccagtaacaattctggatgattacagttctgctgacatctggactgtaacctcttgagatatcctgaagaactatagagctatgttgtttctgaattcctgacctacaaaaattttgagataacaagtgtttttgtttgaagccacaaaattttggggggtaatttgttacacagtagcaggtgattcatacatcttgttagagtttgctcatgttatctgaggcatgaaagatcaatgaatgcttttcccacagttattgaattcacatttgcctattatgcattctcgtatgcacagaaaggtaggagttacttgtgaaggatttcccgcaataattacattcatagggtttttttccagtgtgagttctcatgtgtttcttaacggatgagagaacattaaaggattttccacaatcactgcactcataggatttctctccattatgtattctcctgtgaattgtaagagaaaagctattggtaaaggatttcccacactcattacatgtgtagggtttttctccagtatgagttcttatgtgctgtgtcagattcgacctcctcctgaaggttctcccacaatcgtggcattcgtaagggtactcccctgtatgaatgctatagtgcgaagaaagagatgacctcgtgccgaaagcctttccacactgattacatacataatgaccctcccccgtatgaactctcttgtgccttgtgaagattgactgagtgcggaactcacgaaaacactggttacatttgtacggtttttctccagtgtgaattctcaagtgcggtctgaggtatgaggaattgctgaaggttttcccacagtcactgcattcgtagggtttctccccattgtggattctcttatgaacagtaaggtaagatctgctgctgaaggttttcccacagtcattgcattcatagggtttctccccattgtggattctcttatgaacagcaaggtaagatctactgctgtaggatttcccacattcactgcagccatagggtctttctccagtatgaatcttcctgtgccgtgtaagggaagattttgtgctgaagactttaaaacactgattacattcgttgagtgttgctccaagatgattcctctccattttcatatttctagattgttcttttcgaaaaacatgcagcttaggagttaaccctttggctttaaatggattctccacatctggacaggtacctgagagaattcctctctcttctgtcatcactttatcttcttgctccagctgggagatcagcctaggtttatcaacttggttccccagtgaggccaggttcctgcagttctccagcatcacgtccctgtacagtgtcctttgggcagggtccagcaatgcccactcctcctgggtgaactccacggccacatcctcaaaggtcaccaagccctttagccagcttttcaggagctcattaaccagctctccgccctctgtgtgtccttctcgctgagaggcggcagttgggggcaggacgacagccgccatcctgtgactccgacagcaacagggcagccgggaagcaggacgctcctcctttatcccgcagcgctctcaggacagcaccctgatcatacagaagtccacggatcagtgaggataggtgaaacttgaggctggtttcaacacaaatctgagcttgaattatacttttttcgtggaatgaagcacctctcgcggagaccgaaagattctcccagacgctgcaagcgcggctcttctcacaagac

SEQ ID NO: 16049 - RNA, 4557 nt, Homo sapiens
  source 1..4557: mol_type = other RNA
gctgggattacaggcatgagccatggcgcctggccccactgtacattttcaatactgctcattgacaacttatctttttctttaagtagggagaatgaacattaagaaacagtatttgtgccgggcatggtggctcacgcctgtaatcccagtgctttgggaggccgaggcaggtggatcacgaggtcaggagattgagaccatactggctaacacagtgaaaccccatttctactaaaaatatgaaaaattagccgggcatggtgatgggcacctgtagtcccagctactcgggaggctgaggcaggaggatggcgtgaatctgggaggcagagcttgcagtgagccacaatcgcgccactgcattctagcctggacaacagagcaagactccgtctcaaaaaaaaaaaaaaaaaaaaaaagaaacagtatttgctatattaggacacaaagagaaaacaaccaaaatcacaaagtccatgtactctggcaaaatactattaaattagaaaaaaatatatcaaatattgtctgatttttttttttttgagacagagttgcactcttttgcccaggctggagtgaagtggcatgatcttggctcactgcaacctccatttcccgggttcaagtgattctccttcctcagcctcttgagtagctgggattatagatgcctgccaccacacccggctaatttttgtattttttagtagaagcggggtttcaccatgttggccaggctggtctcaagctccttacctccggtgatctgcccgcctcagcctcccaaaatgctaggtttataggtgtgagccaccacacctggcaaatgtctaatttctattataacaaactagatcactcaggagctgtttggaaatacctttctgaatatttggtgtattgatgttttagaattataataaatacactgtatataaaacgaggtagtaagattttcaggaccactatagccataaatgtttatattaaaagactgaaaatgaacgagctagtggcccaacctacaaatgagacattgatgaaggtaattccacattcatagcacttacaccttttgttctaagttactgcgtggccactcagttaagagatgaggcatcctaacattgattacgttcctagggcttcctctaaatgaattctctcatgcataaagggaggaatcactgaaaatttttctgaaattaatacactcgtgagtattgcatccaaggaacatttacatatttttcctaatataagaggtatcactgaaaacattccctcatcctttatcttaagaagttctggctgagagtggtagctcgttcctgtattcccagcattttgggaggctgaggcaggtggatcacttgagcccaggagtttgagagcagcctgggaaacatggtgaatccccatctttacaaaaactagacaggcatggtggtgcatgcctacagtcccagctacttgggaggctgaggtgggaggatcccttaagcctgggaggcagaggttacaataagccaagattgcaccactgcactacagcctgggcacagatgaaaccctgtctcaaaaaataaattgtataaattgttatcttacactgagttaggttcctaaaaatgtggaaaaatgacattctaatactgatggaattcaatggtttttctagtatgaatctcacttcttaaaaatggagagaatattcaaggcttttatagcataccaaactatactgtcttgtgcttggtaatatgactgtttgtgtcacaggcttttcaacactgtgtatactcaacatattcctctgttgtatgatctccgaaatgtgacttaaggaatgagtgtcccctggttttccatttttgatgccacacacagggtttccccttattgtgagttgtcatgtgactccctgaagccatcactgaaggctttcctacagctactgcattacctgggcagctccccagtagatactttttttttggtagggggaaagtttgagctcaaagttttaccatacagattacactcacaagatttctctctagagtgagttaacctgtgggtgattgaatgctactcccatattgatcagtttagaagttggctgggcatggtggttcatgcctgtaatcccagtacttctggaggccaagatgaaaggactgcttgaacctaggagtttgagactagtctgggcaacatggcaaaaccctccctctagtttaaaaaaaaacaaattagccagacatggtgtcatgcacctgtagtcccagctacattggaggctggggcaggagaattacttgatcccaggaagtagaggctgcagtgagctgtgatcacaccactgcgctccagactgggtgacagagtgagacattgtcttaaaaaaaaaaaaatgagggtcagctgaaggctttcctccactgatttcatggcaagttttccagatggttccaaatgtctactgttcatacctcctgtggtgttcttccacattgtatcaggattggtgtgtatgaccaatgtaacagggacatgaaaacatatctcactgaagctaggtcataaaagacattatgctttctgtgttggctcctttagatcactggctttggggagaagttgcttccataaagaaactcagccctgttgagaggcctacgtgatttggaagcgcagctcccttggaaacagctagcatgcacttgtcgggcttgtaagccatttggaagtggtcccttcaccagtaacaattctggatgattacagttctgctgacatctggactgtaacctcttgagatatcctgaagaactatagagctatgttgtttctgaattcctgacctacaaaaattttgagataacaagtgtttttgtttgaagccacaaaattttggggggtaatttgttacacagtagcaggtgattcatacatcttgttagagtttgctcatgttatctgaggcatgaaagatcaatgaatgcttttcccacagttattgaattcacatttgcctattatgcattctcgtatgcacagaaaggtaggagttacttgtgaaggatttcccgcaataattacattcatagggtttttttccagtgtgagttctcatgtgtttcttaacggatgagagaacattaaaggattttccacaatcactgcactcataggatttctctccattatgtattctcctgtgaattgtaagagaaaagctattggtaaaggatttcccacactcattacatgtgtagggtttttctccagtatgagttcttatgtgctgtgtcagattcgacctcctcctgaaggttctcccacaatcgtggcattcgtaagggtactcccctgtatgaatgctatagtgcgaagaaagagatgacctcgtgccgaaagcctttccacactgattacatacataatgaccctcccccgtatgaactctcttgtgccttgtgaagattgactgagtgcggaactcacgaaaacactggttacatttgtacggtttttctccagtgtgaattctcaagtgcggtctgaggtatgaggaattgctgaaggttttcccacagtcactgcattcgtagggtttctccccattgtggattctcttatgaacagtaaggtaagatctgctgctgaaggttttcccacagtcattgcattcatagggtttctccccattgtggattctcttatgaacagcaaggtaagatctactgctgtaggatttcccacattcactgcagccatagggtctttctccagtatgaatcttcctgtgccgtgtaagggaagattttgtgctgaagactttaaaacactgattacattcgttgagtgttgctccaagatgattcctctccattttcatatttctagattgttcttttcgaaaaacatgcagcttaggagttaaccctttggctttaaatggattctccacatctggacaggtacctgagagaattcctctctcttctgtcatcactttatcttcttgctccagctgggagatcagcctaggtttatcaacttggttccccagtgaggccaggttcctgcagttctccagcatcacgtccctgtacagtgtcctttgggcagggtccagcaatgcccactcctcctgggtgaactccacggccacatcctcaaaggtcaccaagccctttagccagcttttcaggagctcattaaccagctctccgccctctgtgtgtccttctcgctgagaggctgggaacagggaagacagagcggcagttgggggcaggacgacagccgccatcctgtgactccgacagcaacagggcagccgggaagcaggacgctcctcctttatcccgcagcgctctcaggacagcaccctgatcatacagaagtccacggatcagtgaggataggtgaaacttgaggctggtttcaacacaaatctgagcttgaattatacttttttcgtctctcgcggagaccgaaagattctcccagacgctgcaagcgcggctcttctcacaagac

SEQ ID NO: 16050 - RNA, 4569 nt, Homo sapiens
  source 1..4569: mol_type = other RNA
gctgggattacaggcatgagccatggcgcctggccccactgtacattttcaatactgctcattgacaacttatctttttctttaagtagggagaatgaacattaagaaacagtatttgtgccgggcatggtggctcacgcctgtaatcccagtgctttgggaggccgaggcaggtggatcacgaggtcaggagattgagaccatactggctaacacagtgaaaccccatttctactaaaaatatgaaaaattagccgggcatggtgatgggcacctgtagtcccagctactcgggaggctgaggcaggaggatggcgtgaatctgggaggcagagcttgcagtgagccacaatcgcgccactgcattctagcctggacaacagagcaagactccgtctcaaaaaaaaaaaaaaaaaaaaaaagaaacagtatttgctatattaggacacaaagagaaaacaaccaaaatcacaaagtccatgtactctggcaaaatactattaaattagaaaaaaatatatcaaatattgtctgatttttttttttttgagacagagttgcactcttttgcccaggctggagtgaagtggcatgatcttggctcactgcaacctccatttcccgggttcaagtgattctccttcctcagcctcttgagtagctgggattatagatgcctgccaccacacccggctaatttttgtattttttagtagaagcggggtttcaccatgttggccaggctggtctcaagctccttacctccggtgatctgcccgcctcagcctcccaaaatgctaggtttataggtgtgagccaccacacctggcaaatgtctaatttctattataacaaactagatcactcaggagctgtttggaaatacctttctgaatatttggtgtattgatgttttagaattataataaatacactgtatataaaacgaggtagtaagattttcaggaccactatagccataaatgtttatattaaaagactgaaaatgaacgagctagtggcccaacctacaaatgagacattgatgaaggtaattccacattcatagcacttacaccttttgttctaagttactgcgtggccactcagttaagagatgaggcatcctaacattgattacgttcctagggcttcctctaaatgaattctctcatgcataaagggaggaatcactgaaaatttttctgaaattaatacactcgtgagtattgcatccaaggaacatttacatatttttcctaatataagaggtatcactgaaaacattccctcatcctttatcttaagaagttctggctgagagtggtagctcgttcctgtattcccagcattttgggaggctgaggcaggtggatcacttgagcccaggagtttgagagcagcctgggaaacatggtgaatccccatctttacaaaaactagacaggcatggtggtgcatgcctacagtcccagctacttgggaggctgaggtgggaggatcccttaagcctgggaggcagaggttacaataagccaagattgcaccactgcactacagcctgggcacagatgaaaccctgtctcaaaaaataaattgtataaattgttatcttacactgagttaggttcctaaaaatgtggaaaaatgacattctaatactgatggaattcaatggtttttctagtatgaatctcacttcttaaaaatggagagaatattcaaggcttttatagcataccaaactatactgtcttgtgcttggtaatatgactgtttgtgtcacaggcttttcaacactgtgtatactcaacatattcctctgttgtatgatctccgaaatgtgacttaaggaatgagtgtcccctggttttccatttttgatgccacacacagggtttccccttattgtgagttgtcatgtgactccctgaagccatcactgaaggctttcctacagctactgcattacctgggcagctccccagtagatactttttttttggtagggggaaagtttgagctcaaagttttaccatacagattacactcacaagatttctctctagagtgagttaacctgtgggtgattgaatgctactcccatattgatcagtttagaagttggctgggcatggtggttcatgcctgtaatcccagtacttctggaggccaagatgaaaggactgcttgaacctaggagtttgagactagtctgggcaacatggcaaaaccctccctctagtttaaaaaaaaacaaattagccagacatggtgtcatgcacctgtagtcccagctacattggaggctggggcaggagaattacttgatcccaggaagtagaggctgcagtgagctgtgatcacaccactgcgctccagactgggtgacagagtgagacattgtcttaaaaaaaaaaaaatgagggtcagctgaaggctttcctccactgatttcatggcaagttttccagatggttccaaatgtctactgttcatacctcctgtggtgttcttccacattgtatcaggattggtgtgtatgaccaatgtaacagggacatgaaaacatatctcactgaagctaggtcataaaagacattatgctttctgtgttggctcctttagatcactggctttggggagaagttgcttccataaagaaactcagccctgttgagaggcctacgtgatttggaagcgcagctcccttggaaacagctagcatgcacttgtcgggcttgtaagccatttggaagtggtcccttcaccagtaacaattctggatgattacagttctgctgacatctggactgtaacctcttgagatatcctgaagaactatagagctatgttgtttctgaattcctgacctacaaaaattttgagataacaagtgtttttgtttgaagccacaaaattttggggggtaatttgttacacagtagcaggtgattcatacatcttgttagagtttgctcatgttatctgaggcatgaaagatcaatgaatgcttttcccacagttattgaattcacatttgcctattatgcattctcgtatgcacagaaaggtaggagttacttgtgaaggatttcccgcaataattacattcatagggtttttttccagtgtgagttctcatgtgtttcttaacggatgagagaacattaaaggattttccacaatcactgcactcataggatttctctccattatgtattctcctgtgaattgtaagagaaaagctattggtaaaggatttcccacactcattacatgtgtagggtttttctccagtatgagttcttatgtgctgtgtcagattcgacctcctcctgaaggttctcccacaatcgtggcattcgtaagggtactcccctgtatgaatgctatagtgcgaagaaagagatgacctcgtgccgaaagcctttccacactgattacatacataatgaccctcccccgtatgaactctcttgtgccttgtgaagattgactgagtgcggaactcacgaaaacactggttacatttgtacggtttttctccagtgtgaattctcaagtgcggtctgaggtatgaggaattgctgaaggttttcccacagtcactgcattcgtagggtttctccccattgtggattctcttatgaacagtaaggtaagatctgctgctgaaggttttcccacagtcattgcattcatagggtttctccccattgtggattctcttatgaacagcaaggtaagatctactgctgtaggatttcccacattcactgcagccatagggtctttctccagtatgaatcttcctgtgccgtgtaagggaagattttgtgctgaagactttaaaacactgattacattcgttgagtgttgctccaagatgattcctctccattttcatatttctagattgttcttttcgaaaaacatgcagcttaggagttaaccctttggctttaaatggattctccacatctggacaggtacctgagagaattcctctctcttctgtcatcactttatcttcttgctccagctgggagatcagcctaggtttatcaacttggttccccagtgaggccaggttcctgcagttctccagcatcacgtccctgtacagtgtcctttgggcagggtccagcaatgcccactcctcctgggtgaactccacggccacatcctcaaaggtcaccaagccctttagccagcttttcaggagctcattaaccagctctccgccctctgtgtgtccttctcgctgagaggctgggaacagggaagacagagcggcagttgggggcaggacgacagccgccatcctgtgactccgacagcaacagggcagccgggaagcaggacgctcctcctttatcccgcagcgctctcaggacagcaccctgatcatacagaagtccacggatcagtgaggataggtgaaacttgaggctggtttcaacacaaatctgagcttgaattatacttttttcgtggaatgaagcacctctcgcggagaccgaaagattctcccagacgctgcaagcgcggctcttctcacaagac

SEQ ID NO: 16051 - RNA, 3461 nt, Homo sapiens
  source 1..3461: mol_type = other RNA
gctgggattacaggcatgagccatggcgtcacttaaatgtagtgagaggccgggcacagtggctcatgcctgtaatcccagtactttgagaggacgaggctgtcagatcacctaaggtcaggagtttgagaccagcctggccaacatggtgaaaccgtgtctctaaaaaaaatagaaaaaaatatccctgcatggtggtgagtacccgtagtcccagttactcaggaggctgaggcatgagaatcgcttaaacctcggaggcggaggctgcagtgagctgagatggcgccactgcactccagcctgggtgacagagcaagactttgtctctaaatatttaaataaataaatatggccgagcatggtgccttaggcctgtagtcccaacactttgggaggctgaggcaggtggttcatgaggtcaggagcccgagaccagcctggccaagatggtgaaacactgtctctactaaaaatacaaaaattagccagctgtggtggcaggcacctgtaatcccagctacttgggacactgaggcaggagaatcacttgaaactggaagtcagaggttgcagggagccgagattgcaccactgcactctagcctgggcgatggagcaagactccatctcaaataaataaattaataaatacagagcaagattccatcttaaataaataaataaataaacatacacctgtaatcctagcagttcgggaggctaagacaggtcgatcacctgaggtcaggagttcgagaccagcctgaccaatatggcaaaactccatctctactaaaaatacaaaaattagccaggcgttttgacgtgtgcctgtagtcccagctacttgggaggctgagacaggagaattgcttgaacccaagaggtggaggttgcagtgagccaagatctcggctgcacttcagcctgggtgacagagtgagactgtctcaaaaggaataaaaaaaatacaaaataaaaaaaatgtagtaagattgcagagtcgtgccgcggaagcgtgctggtcctatccatgtagtgaaggctgatttcatacacaaatgtcacaagaactttttttctttttcttttttttttgagacggagtatggctctgtcacccaggctggattgcagtggcgcgatctcagctcactacaagctctgcctcccgtgtttatgccgttctcctgcctcagcctcccaagtagctgggactacaggcctgtgcagcagatgcaggggggccactaggcccaggcagtcttgggacttgtgtgtctcctgctgtgcatccatactgggtgctttagaaacggcaggcagaccagaagcccctgttgcaagtgaggacaaagtgtgggaaggccgtgagggtctgcagtccgagatggcctggtcctcaacctgcagtgcactgttgatgcgctggaaggccgcctccttctcccggtccaggtcttcagcagtgacccggtaccccatctctaagggaggtggcagcatcaaaggctcccctcgcctgcgtggcagcaggggaaacttgcatctacggggcctagaggcctgggatctgggggagccacccctgggggcgagtgtctgccctggtgctgtatctgccgtcttttcacactggatgtgacccgaagagacagcctgaggtccgtcctcactcagtgtgtttcaggaactgagggtcagctggcagtgggatgaggctggcccctcttccgctttcgttccgggaggcctcccgtagagctgtaggggctcgagatggcatttcatttggggcacgagctggtccgggaggtctgggatctctggttctgacctctgggcacctgctgcagctgtggctgaggcccagaaatgtgaagggcctccatccactccagtagtgaccccaacgtggggttcagtgtggaggggggaggggctgctgtggcagctgcaggagcagaagtgccacgccttgttcttctcatgcctgcatccatgcttgcagctgggaagggggcaggaatcagcgaggtgacctgggctgagtcctgggaatcagaagaggtggcaggaaggggatctgaggaggagaacagggggcctggtggtctgtgcttcttcccagacacgggagctgtagaggggacctctgcagcagatgctaagggggccagtaggcccaggcagtcttgggacttgtgtgtctcctgctgtgcatccatactggatgctttagaaacagcaggcagaccagaagcccctgttgcaagtgaggacaaagtgtgggaaggccatgagggtctgcagtccgagatggccttgtcctcaacctgcagtgcactgttgatgcgctggaatgccgcctccttctcccggtccaggtcttcaacagtgacccggtaccccagctctaagggaggtggcagcatcaaaggctcccctcgcctgcgtggcagcaggggaaacttgtgtgtactgggcctagaggcctcggatgtggaggagtcattcctgagggtgagtgtctgccctggtgctatatctgctgccttttcacactgggtgtgacctgaagagacagcctgaggcctgtcctcactcactgtctttgaggaactgagggtcagctggcagtgggatgaggctggccccctcctccgctttagccccggcaagcctcccgtggagctgtaggagctggagatggcatttcggttggtgcaggagctcgtccaggaggtctgggatgtctggttatatctgatttctgacctctgggcatggaggtctgtctgcagaggcccgggcctgggcacaaagggagagaggcctccattgtcccgcaggggccgaaatgcagacggtgcatccccggtgacctcggggacccttctctgatcaccaggattctcttggactctagggtccttgtcctgctcaggcatccctgccccgctctccttgagggccctcaacactatcttccctggacacaagtctggggacagccgggtgttgtggaccccaaaggggtgactcccggctcctgggccccacagagagtccatgttctcagtgcagtggctgagctggaggacgccctggaactcggagcacacagcactggcttgctgtggtacctgtgcaatcaaattgaaggcaggatcccaggaaggaacgcagggcttgcaggatcaccgaaaaccttcttagagttgtcttgacaccactgatgtcaagtgtccgggtgcttgtaggatggcctgccactcagtccacgggcaggagcaacggggagatcccacaagcaaagtgaactgggggatgggctgaacgggctccaggcaactgagccctactggcaggtcctcggcctgggcccgaacaggaaggaggggcacagagtgcccaggtaaccgctcctgggagcagtggggaaccgtcggttgctt

SEQ ID NO: 16052 - RNA, 9240 nt, Homo sapiens
  source 1..9240: mol_type = other RNA
gctgggattacaggcatgagccatggctcccagccagcttttaacacttttgattggaaagggccagctttagtcttagcagagcagcaaatgtcagcctcaaggcaacataccaaagtagtaaattattagcctagaacctagaacccagaacccaaaatctaccatctccttcctttaacaatgccctttctgaccatcttcaagaaagttcacccaaaattatgtctttcgcataaataaatttcttatgccactacttttggctaaaatcttttgatggggatgaattactcctctcacatcctctagcttttcctttacaggacttttatgttttgaagaactcattaaatcactaaatttactaaccttttgtgaactagtaagaatgaaagtaacttgtgtataaccaactaatgggatagtttgtgtgtgtgtgtttaaacggatgatttcgctctattttctaaccagaagggccaggaggactagatgatttaactttattatattgtaatatcaaaaatatccttaaaagacactgaaaagatgtttagaaaattcatattcattaaaccatctttctgacctgtatcttcaatttcagatagaaaaaaagggacccacactcttaaactggagagtgcatttagaattacacaaactatcctactatgactcaggaatggattgtgttctggcttactgtgtggtgacaaggccacatctgtcaaaggcaaagaaaacaacatgattgctttttaaattgtattttttctaggttaaaaaaaatcaccgcaaaaccaaaccaaaccaaacaaaaatggctgctgtctaaataagcaggaggcatcagtttattcactgctaccacaaaatttggaaaagcaatttgggttagaggatcacttaattacccccttgaagctagaaagtaagttattcaattttaatctggcttgaaaatgtattatttgcaaaattcaaaaacattctttccagctttacctcaaattcactgtcagcttcaactactgtcattctaattatctcactccaaaagtttggcaggtacatatctgatcaaacacagaatgtgaacatgtgtgcacaggtgaccttatatccccagataaattacttatatcttggactatgtgcaacaggtatcagctcatctctaggttccaacgataaaggaaggcactttggctatctggttctcccatgtatgtacactgggcacatagcagtttgtgcactgggcatacagaaggcactcaacaaatgagtgaaactaaccaaagtcataaaaagctgaatgttttaaaattttttaaaatacagaaacaattattaaactcacatatatgcttaacctgctttctgaattttcatttaaagtcaaacatgaataaatgcatttgttctggggcacacgtttaaccttgtgtcatagcacacatatgctaagctatagtcttgacagtgcagagaagctcctataaattgttggacactgtaatgctctccaagtaggaaaatacaccaagaggatgagcccaacccagagttttatgtgtattaaggagcttggacttgtacattgctctttcccaaccctatttccacagaggatagcattcaagagtttgacttgactttcccagaacgctacaagtttttaagcttgatgtatggtaaacttacatctcaaaagtccagtaagtagttaacttctagttccagaactattactgctgatttaacttgctttaaaagagtatgattctagggtgggcatggtggctcatgactgttatcctagtactttgagaggccaaggcaggaggatcactttgaaactagttcaaaaaccagcctgggcaacaaagtgagagccatctccacaaaaaaaacaaaacaattagccaggcgtgggtggtggtgttatgcacctgtaataccagctacttcgaagtctgaggtgggaggattgcttaagcccaggagtttgaggctgcaatgagctatgatcatgctactgcattctagtctgtgcggcaaagcaagaccctgtctcaaaaaaaacttccagaaaaagaagtatgattctagttggccttggtaaattggtcagttgagggtggaatttgatatagggtagaagttccattcagggaatggaaaatttacaaaggccaaatataaatataaaactgcataataaagacacaaaccaaactgttaacaatggttacctctaaaaagggatgtgggatgatgagggaagggagatctaaaaaggaacttttgtttttactctatattaaaggcacagatcaaatacaagtttgaatttttggtagcatcatgtcctgttatgggagttgctgtcagagttgtataaagacttgttttagtttatcttgtacttttccccatcagttatacctttcctctttttccttcttccctccaataaaaaacgtattctgataaaagaatctgctaaagttaactcctagattttatacactaagcagtcaaccgtcagccaaaagtaatgaacttcaaatacattacaagaggccttctagtttcctgattcacatgcttaaagcagaccctgattctgtctaagcattggcttgcatttaaattctatgatactgactgggcctagtggctcacatctgtaatctcagtactttgggaggctgaagtgggaggaatggttgaggccaggagttcaagaccagcctgggcaacacagcaagacttcccatctctactaaaaatgaaaaatacaaaaattagccaggcatggtggcttacacatgtagtcccagctactcagaaggctgaggcaagaggattgcttgagtccatgagttcaaggatgcagtgaactatcactgagccaccacactccagcctgggtgacacagcgagactgtctcaaaaaaatgaaataaaaaaataaataaatttggatactaatgaaatccacctaacagaccagattccttttcaggtttcatggagtcagaggctattttaaaaaagaaaaaaagaaagaaaaaaaaaagaaaaaggcaagacacatccatagaaatgtgggaggaaataaaatgaaaaagtctgtatttaccaaagagctcctagacacgttggcaagagaaaaggcaaatggcaaaacacatgggtaagacacaatttatgtgaaaatttaaaacccacaacactatgtatttctatatgtaaacatatagatatattaatacatagcaaaaagatatttgaggagtatatactagagaccaatagttactaccatttgggagcactaccaaagggcactttgacaatatatgttttttattcttttcctagaacattttcttacataattaaatacaaaatgaggaactttcatatttctaggaagtaccacatacaatgatttccttaaaatagcttgctactaaagctagagtttagcagataccacttctttctacttttcaacattatactttatccttgctatccctcaccattctctcattgatctacacatgttcaaatgtaaagaaatcaccttagctttttcttaaaatacgtgatagtgaagagatgatacagttgccagaaagtatcaaaatcaagactgagaactggtatagtgggaataaaggccactgaagtaggcaactccacctcctcttgacttgtgcctttaatatgatgcatttgaaaatatgtgcagacttctaaagaaagatgctttaagaataagagacctaactgggtatgctgtgtaacattaactcatcatgtttactcatatatctactgaagagaaaatgttgcagtagaaaggttaatgcgccaaagcagttttccagaaaagcaaaaatgtataaatcctagatagcacaagaactgctaaaggtctatcaattaagtggtatttatttagaagagaagcatttctgcttgaaattgaaaactcttaggagtatttctaaattttttccaatacataacactattaaaatattacaactaggaaaattttgctcaaaattgcaactgttttcttgaaaaggtaaaggccatcagacatatgtgtagcacgaattttggtccagaacaccaaatatattactctgttatagttgattacagataacagaacagcaacatactaaaatcaatgcatattatgaaatcaagtagatgcggttcaataaattccagcttttaactattaaagcctaggtaatgcattttataatttagagaagagtacttagggatctactcagtttatatctttagacattattgtgaggctcctgcgggtcactactactatctatatccttttccagaaaatatcagcatcttaaatggtcacaaattatgtattccctctttgtcacactgaatctacagagaaaactgaaaactctacagtggcaaacaagtcaaaagatgaattctaaaagttaaaggcacagatcaaactacttttagagataacgtaacgggtaattataagagtaaactatactatctgaatatgtaagatcaactatctagaatcctggtagcacttataatacagaaaattgcaaattatataattaaagaaataaacagtatcacaatccatttttaaaatgttcttaatatttggcataatgcatagtttgccttaattagaaactctttgataaaagtaatgtacttttcaaagtgatttaaaaaactgtcaggttgtagttttttatttacttgacttccattctattcctccctatgctctttccctatttttccaattttatctttcactactaaaaacctaaaagtgaagtactactcttcttcttcactttaatgtcaaatataaagtactccactaataacatatggctactattaaaaaaaaaaaagatttcaatgcagtaacagccatagctttagggtattcttaggcaacaccccagacaaaacaaatctgaacacttatatttcatacaataacataatgcttttttcttttcacattactgcttaccccaaaagcatggcaatatacattttcaaaaacaatcttcccctgtaattacaatgaaaaacaagaagcagaatacccatcatcattacagaaacaatgattgtatacttttaacataatattcaggtatttttaatcactatcttaaaccaatttttaattatataagttaactgtatatgcttactggctgaaaaaatactggcacaacctacctactgcttttaatacacaacgtggtaacttgtgtcttctgcctaatagcacaattatcagaaaaagaatgcaaaaggtatattagagaaatgaagaaagcatcagaaaaatttcctcagccttggtttatcatctctttgtctttcctttgtatatatactgaagttgactggtcctctttcattactctattcctacccaaagaccttttgggtttcaaagtgacagcagccatatcatgttgtctattgttgctattgaattagcctcaattacaggcccccactaaaaaggataaagaaatacgtgaggttaagaaagataacacagaaaccaaaggagaaaaaagaaaaaaaaaatatgaagaatagttatgacccaccaataattatctggcaattctggagcagaggttcctatctagctgtttcattaaagtaggatgaaaagctgaagtatagctctccaattatcaggctttagaacgtttttttaaaataaagctcaatttcatctctaactagtttttgtgccttttacgagatggaggtctcagtgttacctaggctggatttgaaatcctggcctcaagtgatcctcctgcctcactctcccaagtagctggccctacaaatgcatgcctctgtgcccagctactctagtttttaaaacatatttcactgtaatgagaaaagcttatttcctatctacttctacaacagtaagaatggaaaagctttcttcactctgtctgaaagagccaggaggtcaaaaacaaagtaccgtgatacccatgattcttgctaccttcccccacccccacataaatactaacttcacaggaaaccaagagactacagagtacaattaccccataaaagaagacaattttagcttatctccctgactcttcccaccccaacttcctcaaaaacacataacagaaaagtctgtgttgagtttagcaaggacaataattaaagaaggtaaagtgaaggctcacagaatgcctcccagtttaagttaaaattccaacatcataacatcagggtgtcaattcattcaacttttaacccatttgagaaggtttaagttattaacttaaaaatatggcagtatttcttttgtaactataatctctttatagcctcttaattgctcatgctaatagctttattacatactactgcttcttataagaagtaaatccaggggccattccattttatcttagacataatatttactagttttccaagcacgacagaaatgaaaaaatatatatattagaacaagaacaatttatgttaatctctacaatctgtgttccttctgcgagcagtgcctgattctactaaaattaacacatttaagttcagtcttatgcttaagaaaaaaaaatctaatgagggactaatttataaagtatacacaaatataattctttaataaatctttccagtgttcactatatctgcattacatgtaatgtttccatccacagaaactcaggatagttcttgtaaaatgaaacagaacattctgtgttcatctctggcaagcaatgaacaaatagaacttgctcacaaaggatctaaaagtgctgcctcaggaacataaactacgtgctatatgaatgagtcttggttaactggctactatctgggatctcttcctctgctcataccactgaacccatctcttataaagcctatgagaaaatgaaagctattgcagaagtgaaattcaacatgagccacccaaattcttctaaggtaaccattctaaagcaaaatcagcagaagtcatctcttctataataacaaacaaaaaacccaaaaggcaaatgctactgctcaatcatcagatgaactcacagaggcaaaaatatgtgacaacagcaataattcaagtaaagtatgtatgaaaatttaaacacgccatgttcaagttaagacagaagtgaaggggagctatgatctttatattagtcaaaaaagctaggcataatcaccaaatgttaattcactttacagtcatcaatgagactattgtatatatttttgcaccttgcgcttgtaaaagcagataaaatatttaatatgtaatttacaatgtattttaccagctcagcatacaggatgtatacagattatatcaaagtagtagacagttacgggcctgtgcaaaccctgcaaaaatagtacttcagatatctgctaattaaaaacaaaaacagtttgctgtttagaagtgatacaatttcaactaccacaaaatacaaagggctgcaaaaatgtaaccattccaacaacatatataagttattaaataaagatttgatttgaaagaatataaatgaagactttaagtaggtcttttctacatgcatattattcctcattaaagaaaaaatatgtaaaaaggccattggtaattgctttgttaacatttgtaggccgggcacggtggctcacgcctgtaatcccagcactttgggaggccgaggcgggcggatcacaaggtcaggagatcgagaccatcctggctaacctggtgaaaccccgtctctactaaaaatacaaaaaattagccgggcgtcgtggtgggcgcctatagtcccagctactcgggaggctgaggcaggagaatggcgtgaacctgggaggtggagcttgcagtgagccgagatcaagccagtgcactccagcctgggtgacagagcgagactccgtctcaaaaaaaaacaaaaaaaaacaaaaaaaaaacaaaaaaaaacatttgtagaaaatgccaattctctggtcacaaactccactaagtttagcacttaaggtctctgcagtgttataaacgtaatttaaaatactgttaattctataattccattggtaaaataatgtgacttggaatatggcagtcttcatgttgagggcaatgatccacagttttgttctgtcttttaatttcttaggcgtgaacagttatccagaagaacagcaccctccaccactggtctgggcttgaggttcatcatcaataatctgtacacctcgccttgcagttcccggctgactagagccattgccttttgctctctcatccacttgtgctgtttctatcatccttttacaaaggtcaagaaagagttcctcaattcctttgttctgtttggctgaagtatgataatgttttgctcccacagattctgcatacgactctgcttcttgaatggaaacatgtctctccttttccaagtctattttattaccaactatacataaacagatttcatttcccaacattttccgtaattctttgacccagttttttaccttctgaaaagaatcttcatctgttatgtcataaactaaaatcgctccatttgaatctctgtagtaaattggacccaatgcatggaatctctcttgacctgccgtatcccatatggcaaggtttactcttttcccaccaatatttaacttctttgttaagaatgatgcctgcagagtggtgatgtgcttgtcgttaaacttgttctcgcagtagcgcagcaccagcgacgtcttccccacgcagccttcccccagcagcaccaccttgaacgagtaggctcggcccgccgccgccgccccgccgccgccgccgccggccgcagccatcccgtcgcttcccggccgcccgagcccgagtgtcgcgccgccctcccgacagccgcggcagcgccttcacagccacggccggctcagcccccaccgccccggccccgccgacccgggcgctgtccccacgccctcctcgggcgaggcctggaagggctgagggaaagtccgagaatgaagggccccagcccaccacgtcaggcaccggaggaaaagcgaagaacgatccctctctgcctccctctaatggcgtctccttcctcctac

SEQ ID NO: 16053 - RNA, 3930 nt, Homo sapiens
  source 1..3930: mol_type = other RNA
gctgggattacaggcatgagccatggggcctggccagggagacttttctatccatgctgcacggcaatcttgtcctccttttgctagaagaaataagactcttggggctaggaagaaccttaaatgtcaaattccattttctcttgtcagatgacaaaagtaaatcagcatttcctttaaaaatcggagcactgactttggtcctattcaaaatagctaccttcaattagaattagggtaaaaaatgattcaccataatgttgtttaactttctctcttttttttttttttcaaattactagaattttattagccaagggatagcagctggaggagaaataacaaaaaaatacatcttaagaatccttaagtacagtgcatatttacaatttaagtgtcatattttagaaggccactgtccatcagctcagtaaatgtaccagcttctaaagccatgatgccataggtccatttgttgatgaaattcctacccactgtcctcgggcatctgactctggtctctgcactggcatcaagagaacgctgctcggtggtttaaggctaacaccttacagggtaacactgtaacactggccctggagccaggtgcttttctccatgaaaacttccaccttggtagctcagccgacatagacaacacacaaagcgcagctctgcacttctgtccttatcttcacacagtgacatccacaccaggtggccaaacagaagagaaggcagaggcccaccaagagctgatgctgcgcagtccttgggggatcatcctccggtctcactggggacgaacccaggttctggagcctctcccctgacagacagcttgtcaccggcacttatgggtcctctgggatttcagacaatacccaacttctgtaggttcagaaagtgctttcaagcaggcagtggcacccacacccggtgggacacacctcctgggtccgaaaccactccatcatgtggctggtgtggccaccgtgcccacaggtcaggcagaaattggacgatccccgcacagccacgtgacagatggcacactggaacgtgaagcctttgcagatggcacactgcgtgccacggacctcactccggcagtggctgcagtacacgccgaactcgatccctttgtgagggtcaggaggacaggagacaaacttcaacacttcagctcgcttctctctcagaccccaacggtagaggatttccccatagcatttcttaaagtcatcaaattgctgggtattggcggggtccaggagccttttatttttatcatgctggtcgcgttctcgctcacggggatcactgtaggtcagactcccaaagcggagctcttctggtgaggattctccccaaggggaggacaagtgctctgcctctcttcccgctatgttccagccgccagtgttgagccctgggtctgacatactggagcaggaaccagaagaggtaaagctaggatatcgactatgggacaccacaagattagaagaacggttaggaaaaggcccaaaggggtttggtagcccctgaggccgagactgggcttcaaacacgctacagagcatcgccagtgtctgaacatcccggagccggcaatagtgagccaacagggactccagcagctgccgcccaaatggatgtcgagcccagggtgtttccaaatctgggtcagatttcggaccaaggcaaagatctgtagctaccgtagccagcgaccaaacctggacaagatcctttcttccaacgagcaaggcagaggcggcattcttctgacatgtttcctgaatatcattcacattcaatatgtacagctctcccagcgatttgtgaacaggcaggaggcaagcaatatcctggatgatgactttcccagcagccttgatctgtcgattgccagagtctgatccctcacgcttacttttccatcgtcttgatttccgctccttgtagtagaaggagctgatggagacctgctctttctcgctgcgagtggggctcccactgtataaacgaaggttcccaggggcctctgtgcggatcttcatgggcgcgatcaagccagtgtgataagcagacaaggctgagagagatctcggagtaggctctgtgggagacaccgcccgatgcattgtcatgggccttgtgaaatataccaggtaacctgctccgcagaacctggccccagaagtcctaggaaagggaatgttggcgtcctggtacgacccgtaagccgtggtcacccgcgcaaacgtcggtaaggggggagtgacagagttggggagtgcaaacgggttgctggaagcgctgtcttcctggttcacaaaggactcaaggcaggagacgagctggcgcaggcagggctccaggcagctctggccacgcttcactttctgcagggctgtgtccttcaggatcttcagcagcttagctttcatggtggatgtgatggttgtggggttaataaactggaaggaaggggcggcgttgtttgggtactgtgcagggaacttcaccagcatcttgacacgatggttgctgcagtgcacagacactgtgcagctcctgtctgccgcatccatctccacattgacattccggatttgcacattgatcagggagaattcctgctgcaaggtctgaggcagccccagttgatctgatttcctctcttccaggagatttctagggggatcttcttttagggcttcttcctccccatggcttgcagtgtgctggtgatctgtatcttcagtgtgcagggtcttctcaggttccggcagaagggaaatactctcaatgaactcatcaacaccatctaatatgtcatttgcacaaagcctctgcatctgggaatccacccgccacattctcaaggtctgatcccgggaccacgtcaccagttgatagtccttggacccttccttctgcttcctccactggaactccaggaccacatcatcatgccccacgaaggtgtggactggggtgttcaagtcaaagacattccacaggagaaggctgttttccctccgcagctggggaaccatcacagtcaccaatccattgctgaaaggtgtgtatctggccttccagacaggcacctggcaaggaagaatattgaggtatttccgaggctggcggtaatcccagaacttcacagaattgtcttgactggaggtagcaagaatgtgctcgctgtctgggtgccagtccaggccatggattttggagaggtgggcggctagatattccactgctgtactgggtttcctcttatcccatatccgcacatcgccgtcatggctggtggcaaggcagttagcattttttttattccatttgacctgggaggcacccgcaacagcagacagtgcaacagtaggtttccttgtgtctttgatatcccaaatgtagatgtaggtgtccacagagctggtaaccaggaggtcaggctcaaacaccgcccagtccaagtcgctgatgacacgagtgtggccttgtaaggttgtgccaacttccccactgccgtctttccacttgtaaaggtctactcgttggttactcgaagccgcaaaatagtgtgcaaagctgtcatgaggattccactgcacagctccaatgtcccatttgctctggcgagagatctttcggtgaccttcgaaaggggcatctagattgacgatgtataagaatctgcggccagaaagcactgcatgctgcccaagacagtccacagacatcgcagttgcctgggagtcacggaactctacaaccacgttttcgctgctccatcgcgccgccatctcccccgcccggccgccgcggccccaggacggcgccctcccaccccgccgtccccagtatcccgggaccgtgcgccccacacagccagagaatcagccccgacac

SEQ ID NO: 16054 - RNA, 1171 nt, Homo sapiens
  source 1..1171: mol_type = other RNA
gctgggattacaggcatgagccatggtgcccagcaaaggtatgttcttgaagttgtcttttttctgagatttatgcaaatggtgcatttggaaaaatagatctgttgggattactattttcaacaagattacttatgtgaaactgactccaagaatctttgggttaaattgatgctcctggaggagagaggccctatttatcctagtatctatgcctggggtcccaactggaacttctccagtttttgcaccgaaaggttcacatcccaggaacccccactcccagggaacttgagttgtcatcttagccatgctgcaggagtgcccagctggaaacgcgtgatgttcatgggaaaaccccaccgtataacatgggttaagctgtgaggtcctttttatatttcagaactttagttgctaaagatagaaagcattaattttattctgtacagttggcctccccagggtgtgctgccctgcagtatcacacactggctgctcagagtccctgggactccactaccacttgatccaagttgagagttccacgagttagccagttaaaacataggatgcccagctaagcttgaattccacataaggtactgaacgacgtccctgaaatgttgcagagagcctggttctctgaagataaggtgttgtaacagtcctgttgaggggagagactgccatcttgtttcagcaactcatatttcaagtgacttttgtcacttgaagctgaagctaatcctgatagaagctgtaaaccacatttctcacagcgggtcaatcgggaaagcacacccactcactacagccattatgggaaaaagggctcgccccttacaggatcctcaactgtggagaggccgggagcccacgcggggcgctggggagtctctcagcaccccaggggttcgggcagggacctgagccgcgccctctctcccgggggtgccctggggtcgaggctgctcggcagagccggcggtcagttcgagccgcgggcccgaacagggctctccccgcggctctctccctcggagtagaaggtgctggacccgaactccagcggagccgcacaacacgtggaggaaaagcgccaggacagctaaccttcccaccttttcaaacctgaaacccggccggctggggacggttggaatgttca

SEQ ID NO: 16055 - RNA, 4607 nt, Homo sapiens
  source 1..4607: mol_type = other RNA
gctgggattacaggcatgagccatgtgcccagtctagaagatctttgacttcaaagaacagataatctagagaccttcacaagtgatcatgttggcactatggtcattacactgagacctataactgggctaggattggttatttacagaaaaaccttgtggtacttaattccaattcatgttaatttatgttatcttgcttaatccttgcaaagcccttttagaggtgggtgttatcccatctataatctgctgcttgtcttagaccaaggaagtgaaagtattcagtccaagcatgctaccatccatttctggtaggtttggtttgtttttagttggctttcctgtttaactgttatttgtcttcctattgaggttagatgtgcattttggaattgcatcattttacatagaaacagctttccagtggagttgactagcatcctaaggacaagtacaaccacttttgaaatagatcatggaaatcacaaagtctgatgttccacaaaatggagtatgatgttatggacactagaaatacaaggtatgggtcattagtaacgctaataacattttcctatagatgacttttaataacactggtttaatgtcaattttttttttttttttttttttttttttttttttttttttttttggagacagggtctccctctgtcacccaggctggttggaatgcaggagttcgaacttggctcactgcaacctctgcctcctaggttcaagtgatcctcccgcctcagtcccccaagtacctgggaccacaggcacacgccaccatgcctggctaatttttgtatattttgtagagatggggtttcaccatattggccaggctggtctcaaattcctggactcaagcagtccatctgcctcagcctcccaaagtgatgggattacaggcgtgagctgctgtgcctggcagaacagtatgaagtgttaacgccaaaatttgttttagctatcatatataaatcataagcatattatttggttggttggtgttagttcattccttcaatcggatgatttaaaataaatgtttttcaagtatcctctgtgatgtatcccaaaggttagcttagaaagaaaagtacttggtgaaccattcctggtgcggagagccctgtttctgctggacttctttggcttgggccgtttcaccatctggggtccttgtggcagtttttgcatctgtagactggttgggtttgtaggtccggccacagctggggcttgggtccaagctgggtgatgtagttattggaggggcattaatcctggaactcagatcgccactcagaaagttctttgcataggaggcgaggttcggcacgctgaccacgcggctgggcacgtcctccaccttctttttcttcatggaaggggtcaaatatcccgggtgaggattgaaagagaaagaccgattccggtgggacatggcactggggaatgctgcgtagtgaaatcttctctcttccgtgagctgcttgatgatgtcctctctctccttcaggcgggtctgcaggcggccaatgagctgaaggtcctcgggcctggacgctcccttccctggcttctctccggaatctttcagttcggcttccagggcagccagccgggcctggagctgggcctgggcactactgaaatctgccaccatggcctgcatctccttccggtgttcctggcgcagtgtctccacctccctggcccgctgggcttgctgagtctcctccaggaacctgcgctggtctcggagcttctgcgcctcctgctgatgctgctccacctccgcgcgcagccgccgcaccgcgtcctggagctgcgcgttctcctcccagagcccgcatccctcgccggaaccctgcccagcagcgcccggtggggagccggcctggcccgggccgccccgctcctctgtggcgattatgtgatccttgctgtctcctggacactggctgctggcttgctgtctgcccagagccctcagctcggcctgcagtgcctccaagtccttctggtgcccagaacaggcagcttgctgctccgacagctcctgtctgagcgactctagcagcagggcctgctgtgcctgcatcctctcacgctcctcctgcagctcttgcctggccttttcctccaaggcctggagctccagtcggtgtgtctggtgttggatctggaggctgtggctggattccttcttcaagcgttcctctgtggccttgagttcctgatgtctggccttctccagcatgcgcagggctctctggtgggaagcctcgagctgggctttcatggcgtggttctgctgagtggtctcctggagctcacgctgcagcttctccctctccaggtccgagagctgcttgagtgcctgcaggtcctccctgtagttgctggtgcactgctccagagcctgctgcatctgtgagacctgggcttgcaatttggccttctggctttgccagtcctcctctagacgctggattttggatgttttctccttcaacaaagagcccagtggaggttgtgggtcacttccctccttgagaagcactttggtcctttcttcttcatcactgctggttccttcttcagctgctaacttatcttgatactcctctcctctcggcgaagtttcatccagcttcaagcatggatcctgggtctccagaatgctgcagtgctggcggcctaattcctggggactttcctcagctcctgtggggcgtgtcttattttgttggataaattcttccagccttaaaacctcaagcagagaattctgaagcttcacattgagggctgctttctcttcttccagctgctttatctccttttctgatttcttcctcacttcctccaactgtgcttctacttccctctgcagtttctttctttcagcctccacggacgagcgaacggatttgatttccacggtgtgcttctttaccaagtcttctagtcgcttcactagctggtctttgagatgtttcttctcctcttctgtctgatgtttgattttacgaaggtcttcttcatattgttgcttcatatattctgtctcagcacttgcctctttcttggtctgcatatctgtgcctcctttcatgcaagggcactccttgagacagctttgatcctgctgaggatgaagattgccggcttccaagtcattctcttcccgcaggactttgttctctgaaactaactcagtcttcatggcatctgtctgctgtgtcccacgacactcctgcagcatcattctgtctttggcaacagccagcttctccccaagtttttttgcagtgcctttcaactctgaattctcctgtcgagcctccttaagctgcacatccaggtcctgaatcctctccttcagcttctgggcgtacttcttcaggtcacttatcttgcggcctctgtgctccaggtctccttccagcttccggacctgagcctgcagggctgactcctggacctggaagttcttgcggaggtccgactccttctcctgccactgccacagggcctggctcaccgactgctgcatggcctgccggatggcctcgttttccctctcgtaggtggcctgcagctcctcggccttgcgggcgtagtccttgctcagctgctggttctccactcgcagccgctgcacctctagcaggacctcctgcatctccgggccctggcctggctccgacttggtttcagggctctcctggggcagccggccctgcggggtagcctcgtggctcgtcaggtgctggagcctcctctcgtagtcagccttgagctccagcatttccctggagagcgtgaggactcgctcggcgtgctctgcctccaccctcagctctctctccttcgtctccagcctgcacgaggccgactcagccagcgcctcctccgtcagcctcttttgcagctccagggcgctctccagggcctggatgcgctgtagaagggcttcctcctctgcgcagccctgttcctgcaggagcctggccttggtctctgccaccgcattctggagctcctcctggtgcgcttcccgcagcgcctccatgctggcctcagcctcatcctggcgggtgttcagggcataaatcaccttggtgagctgggcgatcttcttgcacattttcacgtgcatctggggatcacagtccattctccagccggcgccaccgtcggctttggagccctggcaagtgccgggcgggttaattttgctgttgagagcagaagccatcgctaaaacgcgcccagcactcagactctctcgttttctccctgcccaccgtgtgcacgtgcgtgcgcgcgcgggcgtgcgagcgtgtgggtttctcgggagaggtggcactgcagtcccgtcgcctgcaccgccgcgtggccccagcttcccgaaggtctccgcctcccgggcccacccgcgcgcccaccctttttcctctcctgctggttctctggctggctggctccgcgggcacccgcaccctgcggcgaggcgtcggcgccccgcacgtgccgctggcgatcagtctgcagttccccagccagtgcaggtttcgtgt

SEQ ID NO: 16056 - RNA, 5585 nt, Homo sapiens
  source 1..5585: mol_type = other RNA
gctgggattacaggcatgagccattgcacccagtgggggcagtccctttccacaggtcttgagctccagcacagaacacacttgttctattccgtgaagtatggctcagctgtatttccaacggattcatctttcttgccgatgctacctttttagaggattatacagggagtattcaaggtaagctaaagtaaaactatggaaaaacagctcattaatacattctgagtgttcacagaactgtaggcagtgacacatttttgtcattaattcttgacaatcacatacaccgtaaacctacaggaattccaagaactagaggtctgaggactctgaatcttctgcaagttacatatgatttaagagaaaaagaatcaaccctgtataccttagaaatgaggttacagtattgacttcaagaatataaggctcctactgagtctaaaaagacttcgtttcagttcttttggaatgcaaccctgcagtttaagaataatgggagcacaacttccacaggtaacttctacatttattttataccaaaaaagttatgtgcaacaaataaacattcttacatatttacatttggttttatttaccagttagcaaaacagtgccttaaatctctgataaagagtatttctatctagattaaaggggaaacctgcccagtgaactccattttaaatgactgtttactctggagcttaaagcactagtaagaaatatttctgatggaacatactacacagatcatatacctaataaatacttaggccatgcttaatacagttttataacaaaatatttcaccttttctgggcgaatttgtagtaaaaaatgtttaaccaagtagccggggctcccacccttgccctttttgtttgatggaagggtagttctcacaattagaaaccataagtgctgcctgaggtgtctgaaatgtttcacccatgactgtgtgttagagaaaaagacacgaggacagaaattgcatattaggtcattaggtctttttccccaaataggttaccagaaatcacagtgggtctccttgttggcatctaataatgatcttccaagacaagatctcctgtcactcttggtaccaatctaagttgtgaagtaattgctgaagataactctgtacttttgcaaatagtcttttccaaaactaaatgaaaaacaaaagtcaacaaatagtttttatttttatttttttatttgagacagagtttcactcattgcccaggctggagtgcaatggcgcaactgtggctcactgcaacctccacctactgggttcaagcaattctcctgcctcagcctctggaggagctggcattacaggtgccgccaccatgcccagctaatttttgtatttttagtaaagacagggttccactatgtcggtcaggctgatctcgaacttctgacctcaggtgatccaaccgcctcggcctcccaaagtgctgggattacaggtgtgagccaccatgcccagccagcaaacagttttaatttcactgtagtcttggtcctctttgaatgcagtctctctcttttttttttgggggggggacagtctcgctctgttggccaggctggagtgcagtggcatgatcttgactcactgcaacctctgtctcccgggctcaagcaattctcctccctcagcctcccgagtagctgggattacaggggtgtgccactgcgcctggctaatttttgtatttttagtagagatggggtttcactatgctggccaggctggtcttgaactcctgaccttaggtaatccacccgcctcggcctcccaaagtgctgggattataggcgtgagccaccgtgcccggccgaatgtagtttctttgaatgaaaatagtcaatgctttgaacatcatttgaaagtaatgaatttaaggagaggacacatgtatgaaggaacagtgattctgggcacacagctagttaaacctgagttatttcaccggaaatttacctttagtgagagcaactagctgtaatgcaaaacaaatgaaatcctccaaatcacctagattccctagaatttatcatctaaccccaattcctgttatttcttcaaatgatatttgtgaacatcaagtcaataaatggcttcatttggaacaaatcacttaaaaaagatgaggcatggaattactgctaaaaacaaatgtttcccctcatctgtcctttaacactggtggctagtaatgctgcagtgttcaaatattcagtctaaaacaggcaaaacaatcttctaattttgtaacactggtgattccccccctcttctgggcagaatcggaggtatagaaaggaatctgaattctccagggcaaaaaacacccaattaacacccaccaggattctgttactgagacactggcattacaatgctgttatgacaggcagtacgtgttcctctctcagtgagaaaaagggtattaattcgactgggccataggaatgtggcaaaagtttttatacaactgaaacagtggtttccccgaggcttagaaaagcaaaggaaaaactggaagggtctggctgaccattttgccatgttttctcaggtaagagttgaagacatttgcaagaatgcaacatcaagacaagctttaactatactctgttgattgatacaaaataggatgaaaaaccattggatattgggacacgaggaacttgtttagcacaaccgatgtcatgtataccacagttttaaccattaggccatttccactgtagcttagaaaaaagaaccagaggactgccttggtagagctggatgcgctgctacaagatggcctcactgtacagccctcaaacgtgaggacttctttctccatagacaccagatggccaatcagtactttctagagttctttaactacttcagaatgcaagaacagtacatacatactccaacagccattgaaagattcacattcatgggaaaacacaagtcttgatgaaatcttgacttaagctctcttttaagaaactggttgaaactggtgaaaagttcattatgatttggacttgatacctgcctcgggccagaagacctacgttgcatcaattctgagtcagttggaagctacggaattgttgctgactctacacatttgagtttacagagcagagcccgtcccctcccttcaaagagaaggcaaataaagcactcaagagatactggtctcattgactattttcaacataaaatgattaatcaggttggaagcaaaaacattactgctgcttctcaaccagaggattaagtgatcacacaggacccttctgcagagtgcaggttttctacctgacggtgaagaaaggagggaaggacacttcttctgcccaaggtcaacacacaaaatatttggtttgagatttaagacagaaggcacttttaacattctgatatcagatgttaaccatacaaacatcctgtcacaatttcatttgggtgtactcaaatccccttacaaaagtcttcttactgcatgtgtgtcattatgagagcagtggcgacatgagcagatttagccttgagatgtgtctacctgttgctattctcccgatgaagcaaactgggcagcatgtcagccctgaaggttacaaatccagtatttgactgcaaaacaattaaattagacatctgagtggttagtgcagaaagaaacaattagcaagaacactggctcccactccggagcgatggggcttggactggtcttttccatcataatactctttgcttgactggcaccaacgttaaggaaaaatatctgcatgaaaattcaactagtggaagaaactttacctaaaaatgccatgtttatatttccagcttttctccaaagaaaaatacccattttcccatccttagtgtctgaaggccttggacttgaaggtctggccacatgactcattctgtaaggttaacaactggcccagttttatgactgaacacaaactggacttgaacgttccaattcaattttttcctttcagaagagggagatgaaagggaaccgaccaccctattattattttttttgccctattatttgctgcaaccacggctgccagtacttttcacaagatgctgtgtataggctattttcactatctcctcagtcaacgctgagctgacagttcttcagtgctacactccaactaaactgtacagtaagttctgcagaaatggatctaatatttctacctttatttacaaatatcacaaatggattctagttgaatctacatgtttaaatccatcggctaaaaacatattacatattgtaaacatggcaatatttaatacagtatctattctagaatattttcatgtcatgatcacatttgttatacctgaaattgaatttatacacattaaagaattactagcaatggttgctcactttacaattgagggcagggggctagggctacattttatcatttcagaaacacttcaaagtaaagttaaagcttgtctttgattggctcggcgtatcctttttgtatccatatttaaaatgaagactgacacagaaaatagcgagggccccttctaatttaccggatttttaaaaatcagtttgagattcttagggaaagtgtctgttgtgaataataataataataataataataaaaacctgctgcaaaataaactgaatggaaaggggcttgagactgttagggtggagtctgtcgggcgtcagtcctgcttgggttgcagctgccgcttccaggcctcgttcaagtaaactagtcgtttgtagttgataatgagaagaaggaagttcagcacgtacgtgacgatgcagatgatgcagaactccttcagcacaaagtacagaatgtaggccaggtacagggaccccacgaccgacatgatggaggacgtcatgaggatcaaagccgccacagcgcttgctgtcatgccaagtaataactgtagtatataaaatataagtccaaagacactgtttggctggtttaatacaccatcctttccaaaaatggaacccaaaagaccaaatcctcgaccccatctggaggcaagggcggcggagcacttcacccagggccccaggtcgcagagggcccggtgctcggggtcccgctccttctcccgctccacgtggtaggcgtagatggagagcaggattccggcagcgcacactgcataccgggccacccgctcccaccgcggcaccgacactcttagcaggacgggagccgccatcttcccgccgccgccgccgccgcctccctccgcctccacctcagccgccgccgcccgtcggggcccgacccagccgccaccgccgccaccgccgcctccgccgccgccgccaccaccgccgccgccgccgccgcgccccattggctcggtggcctgctccgggccccgcccccacaggcgcgcggcccaaccgccccaaaaggagtgaggcggacggggcggggaaggcgcgcgcgggcgcggagggagggggtggagtgcgcaacggccgaagaggccggatcggcgggcggagact

SEQ ID NO: 16057 - RNA, 5215 nt, Homo sapiens
  source 1..5215: mol_type = other RNA
gctgggattacaggcatgagccattgcacccagtgggggcagtccctttccacaggtcttgagctccagcacagaacacacttgttctattccgtgaagtatggctcagctgtatttccaacggattcatctttcttgccgatgctacctttttagaggattatacagggagtattcaaggtaagctaaagtaaaactatggaaaaacagctcattaatacattctgagtgttcacagaactgtaggcagtgacacatttttgtcattaattcttgacaatcacatacaccgtaaacctacaggaattccaagaactagaggtctgaggactctgaatcttctgcaagttacatatgatttaagagaaaaagaatcaaccctgtataccttagaaatgaggttacagtattgacttcaagaatataaggctcctactgagtctaaaaagacttcgtttcagttcttttggaatgcaaccctgcagtttaagaataatgggagcacaacttccacaggtaacttctacatttattttataccaaaaaagttatgtgcaacaaataaacattcttacatatttacatttggttttatttaccagttagcaaaacagtgccttaaatctctgataaagagtatttctatctagattaaaggggaaacctgcccagtgaactccattttaaatgactgtttactctggagcttaaagcactagtaagaaatatttctgatggaacatactacacagatcatatacctaataaatacttaggccatgcttaatacagttttataacaaaatatttcaccttttctgggcgaatttgtagtaaaaaatgtttaaccaagtagccggggctcccacccttgccctttttgtttgatggaagggtagttctcacaattagaaaccataagtgctgcctgaggtgtctgaaatgtttcacccatgactgtgtgttagagaaaaagacacgaggacagaaattgcatattaggtcattaggtctttttccccaaataggttaccagaaatcacagtgggtctccttgttggcatctaataatgatcttccaagacaagatctcctgtcactcttggtaccaatctaagttgtgaagtaattgctgaagataactctgtacttttgcaaatagtcttttccaaaactaaatgaaaaacaaaagtcaacaaatagtttttatttttatttttttatttgagacagagtttcactcattgcccaggctggagtgcaatggcgcaactgtggctcactgcaacctccacctactgggttcaagcaattctcctgcctcagcctctggaggagctggcattacaggtgccgccaccatgcccagctaatttttgtatttttagtaaagacagggttccactatgtcggtcaggctgatctcgaacttctgacctcaggtgatccaaccgcctcggcctcccaaagtgctgggattacaggtgtgagccaccatgcccagccagcaaacagttttaatttcactgtagtcttggtcctctttgaatgcagtctctctcttttttttttgggggggggacagtctcgctctgttggccaggctggagtgcagtggcatgatcttgactcactgcaacctctgtctcccgggctcaagcaattctcctccctcagcctcccgagtagctgggattacaggggtgtgccactgcgcctggctaatttttgtatttttagtagagatggggtttcactatgctggccaggctggtcttgaactcctgaccttaggtaatccacccgcctcggcctcccaaagtgctgggattataggcgtgagccaccgtgcccggccgaatgtagtttctttgaatgaaaatagtcaatgctttgaacatcatttgaaagtaatgaatttaaggagaggacacatgtatgaaggaacagtgattctgggcacacagctagttaaacctgagttatttcaccggaaatttacctttagtgagagcaactagctgtaatgcaaaacaaatgaaatcctccaaatcacctagattccctagaatttatcatctaaccccaattcctgttatttcttcaaatgatatttgtgaacatcaagtcaataaatggcttcatttggaacaaatcacttaaaaaagatgaggcatggaattactgctaaaaacaaatgtttcccctcatctgtcctttaacactggtggctagtaatgctgcagtgttcaaatattcagtctaaaacaggcaaaacaatcttctaattttgtaacactggtgattccccccctcttctgggcagaatcggaggtatagaaaggaatctgaattctccagggcaaaaaacacccaattaacacccaccaggattctgttactgagacactggcattacaatgctgttatgacaggcagtacgtgttcctctctcagtgagaaaaagggtattaattcgactgggccataggaatgtggcaaaagtttttatacaactgaaacagtggtttccccgaggcttagaaaagcaaaggaaaaactggaagggtctggctgaccattttgccatgttttctcaggtaagagttgaagacatttgcaagaatgcaacatcaagacaagctttaactatactctgttgattgatacaaaataggatgaaaaaccattggatattgggacacgaggaacttgtttagcacaaccgatgtcatgtataccacagttttaaccattaggccatttccactgtagcttagaaaaaagaaccagaggactgccttggtagagctggatgcgctgctacaagatggcctcactgtacagccctcaaacgtgaggacttctttctccatagacaccagatggccaatcagtactttctagagttctttaactacttcagaatgcaagaacagtacatacatactccaacagccattgaaagattcacattcatgggaaaacacaagtcttgatgaaatcttgacttaagctctcttttaagaaactggttgaaactggtgaaaagttcattatgatttggacttgatacctgcctcgggccagaagacctacgttgcatcaattctgagtcagttggaagctacggaattgttgctgactctacacatttgagtttacagagcagagcccgtcccctcccttcaaagagaaggcaaataaagcactcaagagatactggtctcattgactattttcaacataaaatgattaatcaggttggaagcaaaaacattactgctgcttctcaaccagaggattaagtgatcacacaggacccttctgcagagtgcaggttttctacctgacggtgaagaaaggagggaaggacacttcttctgcccaaggtcaacacacaaaatatttggtttgagatttaagacagaaggcacttttaacattctgatatcagatgttaaccatacaaacatcctgtcacaatttcatttgggtgtactcaaatccccttacaaaagtcttcttactgcatgtgtgtcattatgagagcagtggcgacatgagcagatttagccttgagatgtgtctacctgttgctattctcccgatgaagcaaactgggcagcatgtcagccctgaaggttacaaatccagtatttgactgcaaaacaattaaattagacatctgagtggttagtgcagaaagaaacaattagcaagaacactggctcccactccggagcgatggggcttggactggtcttttccatcataatactctttgcttgactggcaccaacgttaaggaaaaatatctgcatgaaaattcaactagtggaagaaactttacctaaaaatgccatgtttatatttccagcttttctccaaagaaaaatacccattttcccatccttagtgtctgaaggccttggacttgaaggtctggccacatgactcattctgtaaggttaacaactggcccagttttatgactgaacacaaactggacttgaacgttccaattcaattttttcctttcagaagagggagatgaaagggaaccgaccaccctattattattttttttgccctattatttgctgcaaccacggctgccagtacttttcacaagatgctgtgtataggctattttcactatctcctcagtcaacgctgagctgacagttcttcagtgctacactccaactaaactgtacagtaagttctgcagaaatggatctaatatttctacctttatttacaaatatcacaaatggattctagttgaatctacatgtttaaatccatcggctaaaaacatattacatattgtaaacatggcaatatttaatacagtatctattctagaatattttcatgtcatgatcacatttgttatacctgaaattgaatttatacacattaaagaattactagcaatggttgctcactttacaattgagggcagggggctagggctacattttatcatttcagaaacacttcaaagtaaagttaaagcttgtctttgattggctcggcgtatcctttttgtatccatatttaaaatgaagactgacacagaaaatagcgagggccccttctaatttaccggatttttaaaaatcagtttgagattcttagggaaagtgtctgttgtgaataataataataataataataataaaaacctgctgcaaaataaactgaatggaaaggggcttgagactgttagggtggagtctgtcgggcgtcagtcctgcttgggttgcagctgccgcttccaggcctcgttcaagtaaactagtcgtttgtagttgataatgagaagaaggaagttcagcacgtacgtgacgatgcagatgatgcagaactccttcagcacaaagtacagaatgtaggccaggtacagggaccccacgaccgacatgatggaggacgtcatgaggatcaaagccgccacagcgcttgctgtcatgccaagtaataactgtagtatataaaatataagtccaaagacactgtttggctggtttaatacaccatcctttccaaaaatggaacccaaaagaccaaatcctcgaccccatttccactgctgctggcaggcctgaggtcctctctggctgttggctggagacatcatttcctgtccacttgcacctcttggtaagaagcggcaggcttgtttcatcatttagttgatgaactt

SEQ ID NO: 16058 - RNA, 5475 nt, Homo sapiens
  source 1..5475: mol_type = other RNA
gctgggattacaggcatgagccattgcacccagtgggggcagtccctttccacaggtcttgagctccagcacagaacacacttgttctattccgtgaagtatggctcagctgtatttccaacggattcatctttcttgccgatgctacctttttagaggattatacagggagtattcaaggtaagctaaagtaaaactatggaaaaacagctcattaatacattctgagtgttcacagaactgtaggcagtgacacatttttgtcattaattcttgacaatcacatacaccgtaaacctacaggaattccaagaactagaggtctgaggactctgaatcttctgcaagttacatatgatttaagagaaaaagaatcaaccctgtataccttagaaatgaggttacagtattgacttcaagaatataaggctcctactgagtctaaaaagacttcgtttcagttcttttggaatgcaaccctgcagtttaagaataatgggagcacaacttccacaggtaacttctacatttattttataccaaaaaagttatgtgcaacaaataaacattcttacatatttacatttggttttatttaccagttagcaaaacagtgccttaaatctctgataaagagtatttctatctagattaaaggggaaacctgcccagtgaactccattttaaatgactgtttactctggagcttaaagcactagtaagaaatatttctgatggaacatactacacagatcatatacctaataaatacttaggccatgcttaatacagttttataacaaaatatttcaccttttctgggcgaatttgtagtaaaaaatgtttaaccaagtagccggggctcccacccttgccctttttgtttgatggaagggtagttctcacaattagaaaccataagtgctgcctgaggtgtctgaaatgtttcacccatgactgtgtgttagagaaaaagacacgaggacagaaattgcatattaggtcattaggtctttttccccaaataggttaccagaaatcacagtgggtctccttgttggcatctaataatgatcttccaagacaagatctcctgtcactcttggtaccaatctaagttgtgaagtaattgctgaagataactctgtacttttgcaaatagtcttttccaaaactaaatgaaaaacaaaagtcaacaaatagtttttatttttatttttttatttgagacagagtttcactcattgcccaggctggagtgcaatggcgcaactgtggctcactgcaacctccacctactgggttcaagcaattctcctgcctcagcctctggaggagctggcattacaggtgccgccaccatgcccagctaatttttgtatttttagtaaagacagggttccactatgtcggtcaggctgatctcgaacttctgacctcaggtgatccaaccgcctcggcctcccaaagtgctgggattacaggtgtgagccaccatgcccagccagcaaacagttttaatttcactgtagtcttggtcctctttgaatgcagtctctctcttttttttttgggggggggacagtctcgctctgttggccaggctggagtgcagtggcatgatcttgactcactgcaacctctgtctcccgggctcaagcaattctcctccctcagcctcccgagtagctgggattacaggggtgtgccactgcgcctggctaatttttgtatttttagtagagatggggtttcactatgctggccaggctggtcttgaactcctgaccttaggtaatccacccgcctcggcctcccaaagtgctgggattataggcgtgagccaccgtgcccggccgaatgtagtttctttgaatgaaaatagtcaatgctttgaacatcatttgaaagtaatgaatttaaggagaggacacatgtatgaaggaacagtgattctgggcacacagctagttaaacctgagttatttcaccggaaatttacctttagtgagagcaactagctgtaatgcaaaacaaatgaaatcctccaaatcacctagattccctagaatttatcatctaaccccaattcctgttatttcttcaaatgatatttgtgaacatcaagtcaataaatggcttcatttggaacaaatcacttaaaaaagatgaggcatggaattactgctaaaaacaaatgtttcccctcatctgtcctttaacactggtggctagtaatgctgcagtgttcaaatattcagtctaaaacaggcaaaacaatcttctaattttgtaacactggtgattccccccctcttctgggcagaatcggaggtatagaaaggaatctgaattctccagggcaaaaaacacccaattaacacccaccaggattctgttactgagacactggcattacaatgctgttatgacaggcagtacgtgttcctctctcagtgagaaaaagggtattaattcgactgggccataggaatgtggcaaaagtttttatacaactgaaacagtggtttccccgaggcttagaaaagcaaaggaaaaactggaagggtctggctgaccattttgccatgttttctcaggtaagagttgaagacatttgcaagaatgcaacatcaagacaagctttaactatactctgttgattgatacaaaataggatgaaaaaccattggatattgggacacgaggaacttgtttagcacaaccgatgtcatgtataccacagttttaaccattaggccatttccactgtagcttagaaaaaagaaccagaggactgccttggtagagctggatgcgctgctacaagatggcctcactgtacagccctcaaacgtgaggacttctttctccatagacaccagatggccaatcagtactttctagagttctttaactacttcagaatgcaagaacagtacatacatactccaacagccattgaaagattcacattcatgggaaaacacaagtcttgatgaaatcttgacttaagctctcttttaagaaactggttgaaactggtgaaaagttcattatgatttggacttgatacctgcctcgggccagaagacctacgttgcatcaattctgagtcagttggaagctacggaattgttgctgactctacacatttgagtttacagagcagagcccgtcccctcccttcaaagagaaggcaaataaagcactcaagagatactggtctcattgactattttcaacataaaatgattaatcaggttggaagcaaaaacattactgctgcttctcaaccagaggattaagtgatcacacaggacccttctgcagagtgcaggttttctacctgacggtgaagaaaggagggaaggacacttcttctgcccaaggtcaacacacaaaatatttggtttgagatttaagacagaaggcacttttaacattctgatatcagatgttaaccatacaaacatcctgtcacaatttcatttgggtgtactcaaatccccttacaaaagtcttcttactgcatgtgtgtcattatgagagcagtggcgacatgagcagatttagccttgagatgtgtctacctgttgctattctcccgatgaagcaaactgggcagcatgtcagccctgaaggttacaaatccagtatttgactgcaaaacaattaaattagacatctgagtggttagtgcagaaagaaacaattagcaagaacactggctcccactccggagcgatggggcttggactggtcttttccatcataatactctttgcttgactggcaccaacgttaaggaaaaatatctgcatgaaaattcaactagtggaagaaactttacctaaaaatgccatgtttatatttccagcttttctccaaagaaaaatacccattttcccatccttagtgtctgaaggccttggacttgaaggtctggccacatgactcattctgtaaggttaacaactggcccagttttatgactgaacacaaactggacttgaacgttccaattcaattttttcctttcagaagagggagatgaaagggaaccgaccaccctattattattttttttgccctattatttgctgcaaccacggctgccagtacttttcacaagatgctgtgtataggctattttcactatctcctcagtcaacgctgagctgacagttcttcagtgctacactccaactaaactgtacagtaagttctgcagaaatggatctaatatttctacctttatttacaaatatcacaaatggattctagttgaatctacatgtttaaatccatcggctaaaaacatattacatattgtaaacatggcaatatttaatacagtatctattctagaatattttcatgtcatgatcacatttgttatacctgaaattgaatttatacacattaaagaattactagcaatggttgctcactttacaattgagggcagggggctagggctacattttatcatttcagaaacacttcaaagtaaagttaaagcttgtctttgattggctcggcgtatcctttttgtatccatatttaaaatgaagactgacacagaaaatagcgagggccccttctaatttaccggatttttaaaaatcagtttgagattcttagggaaagtgtctgttgtgaataataataataataataataataaaaacctgctgcaaaataaactgaatggaaaggggcttgagactgttagggtggagtctgtcgggcgtcagtcctgcttgggttgcagctgccgcttccaggcctcgttcaagtaaactagtcgtttgtagttgataatgagaagaaggaagttcagcacgtacgtgacgatgcagatgatgcagaactccttcagcacaaagtacagaatgtaggccaggtacagggaccccacgaccgacatgatggaggacgtcatgaggatcaaagccgccacagcgcttgctgtcatgcctggaggcaagggcggcggagcacttcacccagggccccaggtcgcagagggcccggtgctcggggtcccgctccttctcccgctccacgtggtaggcgtagatggagagcaggattccggcagcgcacactgcataccgggccacccgctcccaccgcggcaccgacactcttagcaggacgggagccgccatcttcccgccgccgccgccgccgcctccctccgcctccacctcagccgccgccgcccgtcggggcccgacccagccgccaccgccgccaccgccgcctccgccgccgccgccaccaccgccgccgccgccgccgcgccccattggctcggtggcctgctccgggccccgcccccacaggcgcgcggcccaaccgccccaaaaggagtgaggcggacggggcggggaaggcgcgcgcgggcgcggagggagggggtggagtgcgcaacggccgaagaggccggatcggcgggcggagact

SEQ ID NO: 16059 - RNA, 1848 nt, Homo sapiens
  source 1..1848: mol_type = other RNA
gctgggattacaggcatgagccattgcacccggccacaattatttatatttattttactttattttatttatttttgagagggggtcttgctctgtcgccaagctggagtacagttgctcaatctcagctcactgcaacctacacttgccaggttcaagagattctcctgcctcagcctcccgagtagctgggactacagttgcgcaccgccacgcccagctaatttttgtatttttactagagatggggtttcaccatgtttgccaggatggtctcaatctgttgacctcgtgatctgcctgtctcggcctcccgaagttctgggattacaggcatgaaccactgtacccggtcgtattagctatttaaaaactcagacagctaacatttaaataaatccctgctgtctgggaatgatgtctgaatgaatattgtgaatacatatgctaatttataccatattaagattctaaacaatacagctatttaatatatcttgataactggtatttgaaaataagtctatttttctgggtagtcttttggagaaagtgcactgaatatagtttccagtcatatgctactttcttaacttgtacttatctaaacatcttctcatcaggagagagttcaatagtactcgaaccaaaagtctagtgagtctgacttctccaatccccaattttggtttgcatgtccacttacaaccatcatttctctgcaaattttccacttagtctatcaaaaatcagtgctctgaaagttctctaaaagatgcagttttttggagtctctgaatgatgacagcattctgtaaatctgcttcttccagtgtgagtgtctcatctagcaacctgaggacaggaagagctgttgccagggaaaacggaggacttctttgagatccttggtatttttcaatgaagtctttgatatggcttactctatgagtaatgttaaatttctggacaatcctttttccattggccaaccagatctgtatattagtaatgggttccaagttgttcagtggaacagcagacaaattatttttattttcaacttcaatattctttgctttagaaacaatttttggtgtggcacttcctagtctgtgaccctgtcctgaaaagggctggaacacaggcttcgtagacaaacatatttcatttttcttgtcttcaactttaacgtccacctcttctttatcaaaaattccctgtaattctgaaggtaattccccctttttgatggagttcaaaaactgctgactggcaccatcggaataacttctgaaatcgtcgttgacggtgaatccgtttttccataattttatatttacatctaccattcttcttttatacttttgaggttatctacgtctttcattctctttcgccttacaagttccagataccgcccagatgaattttttttttatcacagctgtcattctcatttctacaggcatgaaaagtgcgactcaagttcagtgtcttgcctcgggtagcttggggattcccagtcagctcctcgcgccttcgtcgccgctccccttccaccccgcgccttcgccggccgtcccctgctccatccaggccacgggggtgacggtggggtctggggcattcaggcctggctgggcatgagggcttcaggcccaattccacgcccgaactcgtcctgattagtctggcttttctggtcgccccagccctgcggtcggggagagctggaaaccaccgagctgacagcctagagcgtcgctccccggccgccgagcgctgacgccgcgccgggggcggggcagctggaggcggcagggagaggagcgagcagccgggaag

SEQ ID NO: 16060 - RNA, 1604 nt, Homo sapiens
  source 1..1604: mol_type = other RNA
gctgggattacaggcatgagccattgcacccggccacaattatttatatttattttactttattttatttatttttgagagggggtcttgctctgtcgccaagctggagtacagttgctcaatctcagctcactgcaacctacacttgccaggttcaagagattctcctgcctcagcctcccgagtagctgggactacagttgcgcaccgccacgcccagctaatttttgtatttttactagagatggggtttcaccatgtttgccaggatggtctcaatctgttgacctcgtgatctgcctgtctcggcctcccgaagttctgggattacaggcatgaaccactgtacccggtcgtattagctatttaaaaactcagacagctaacatttaaataaatccctgctgtctgggaatgatgtctgaatgaatattgtgaatacatatgctaatttataccatattaagattctaaacaatacagctatttaatatatcttgataactggtatttgaaaataagtctatttttctgggtagtcttttggagaaagtgcactgaatatagtttccagtcatatgctactttcttaacttgtacttatctaaacatcttctcatcaggagagagttcaatagtactcgaaccaaaagtctagtgagtctgacttctccaatccccaattttggtttgcatgtccacttacaaccatcatttctctgcaaattttccacttagtctatcaaaaatcagtgctctgaaagttctctaaaagatgcagttttttggagtctctgaatgatgacagcattctgtaaatctgcttcttccagtgtgagtgtctcatctagcaacctgaggacaggaagagctgttgccagggaaaacggaggacttctttgagatccttggtatttttcaatgaagtctttgatatggcttactctatgagtaatgttaaatttctggacaatcctttttccattggccaaccagatctgtatattagtaatgggttccaagttgttcagtggaacagcagacaaattatttttattttcaacttcaatattctttgctttagaaacaatttttggtgtggcacttcctagtctgtgaccctgtcctgaaaagggctggaacacaggcttcgtagacaaacatatttcatttttcttgtcttcaactttaacgtccacctcttctttatcaaaaattccctgtaattctgaaggtaattccccctttttgatggagttcaaaaactgctgactggcaccatcggaataacttctgaaatcgtcgttgacggtgaatccgtttttccataattttatatttacatctaccattcttcttttatacttttgaggttatctacgtctttcattctctttcgccttactccgggcacggcctcccggcctcggcctcactcagctcaggcaccgcaggcaccgtttggccgcgggctccgtttggctggagcccttcagagccggagcgccgccgccccagaccgcctcaggttccgcggccgcgccgctgagatcccgccagcctctctcggtcttcgccaggcgcccaagcgcgcgccgacgccg

SEQ ID NO: 16061 - RNA, 1987 nt, Homo sapiens
  source 1..1987: mol_type = other RNA
gctgggattacaggcatgagccattgcacccggccacaattatttatatttattttactttattttatttatttttgagagggggtcttgctctgtcgccaagctggagtacagttgctcaatctcagctcactgcaacctacacttgccaggttcaagagattctcctgcctcagcctcccgagtagctgggactacagttgcgcaccgccacgcccagctaatttttgtatttttactagagatggggtttcaccatgtttgccaggatggtctcaatctgttgacctcgtgatctgcctgtctcggcctcccgaagttctgggattacaggcatgaaccactgtacccggtcgtattagctatttaaaaactcagacagctaacatttaaataaatccctgctgtctgggaatgatgtctgaatgaatattgtgaatacatatgctaatttataccatattaagattctaaacaatacagctatttaatatatcttgataactggtatttgaaaataagtctatttttctgggtagtcttttggagaaagtgcactgaatatagtttccagtcatatgctactttcttaacttgtacttatctaaacatcttctcatcaggagagagttcaatagtactcgaaccaaaagtctagtgagtctgacttctccaatccccaattttggtttgcatgtccacttacaaccatcatttctctgcaaattttccacttagtctatcaaaaatcagtgctctgaaagttctctaaaagatgcagttttttggagtctctgaatgatgacagcattctgtaaatctgcttcttccagtgtgagtgtctcatctagcaacctgaggacaggaagagctgttgccagggaaaacggaggacttctttgagatccttggtatttttcaatgaagtctttgatatggcttactctatgagtaatgttaaatttctggacaatcctttttccattggccaaccagatctgtatattagtaatgggttccaagttgttcagtggaacagcagacaaattatttttattttcaacttcaatattctttgctttagaaacaatttttggtgtggcacttcctagtctgtgaccctgtcctgaaaagggctggaacacaggcttcgtagacaaacatatttcatttttcttgtcttcaactttaacgtccacctcttctttatcaaaaattccctgtaattctgaaggtaattccccctttttgatggagttcaaaaactgctgactggcaccatcggaataacttctgaaatcgtcgttgacggtgaatccgtttttccataattttatatttacatctacctgtttcttctgttcagcgggagacacacatttggaactaaccttctgagcttcctcaaaaaggctatcaacaaaatattcacaatttgattgttgattattaccaagaggttgattatcagatcctgtttcacaaacccattcttcttttatacttttgaggttatctacgtctttcattctctttcgccttacaagttccagataccgcccagatgaattttttttttatcacagctgtcattctcatttctacaggcatgaaaagtgcgactcaagttcagtgtcttgcctcgggtagcttggggattcccagtcagctcctcgcgccttcgtcgccgctccccttccaccccgcgccttcgccggccgtcccctgctccatccaggccacgggggtgacggtggggtctggggcattcaggcctggctgggcatgagggcttcaggcccaattccacgcccgaactcgtcctgattagtctggcttttctggtcgccccagccctgcggtcggggagagctggaaaccaccgagctgacagcctagagcgtcgctccccggccgccgagcgctgacgccgcgccgggggcggggcagctggaggcggcagggagaggagcgagcagccgggaag

SEQ ID NO: 16062 - RNA, 1729 nt, Homo sapiens
  source 1..1729: mol_type = other RNA
gctgggattacaggcatgagccattgcacccggccacaattatttatatttattttactttattttatttatttttgagagggggtcttgctctgtcgccaagctggagtacagttgctcaatctcagctcactgcaacctacacttgccaggttcaagagattctcctgcctcagcctcccgagtagctgggactacagttgcgcaccgccacgcccagctaatttttgtatttttactagagatggggtttcaccatgtttgccaggatggtctcaatctgttgacctcgtgatctgcctgtctcggcctcccgaagttctgggattacaggcatgaaccactgtacccggtcgtattagctatttaaaaactcagacagctaacatttaaataaatccctgctgtctgggaatgatgtctgaatgaatattgtgaatacatatgctaatttataccatattaagattctaaacaatacagctatttaatatatcttgataactggtatttgaaaataagtctatttttctgggtagtcttttggagaaagtgcactgaatatagtttccagtcatatgctactttcttaacttgtacttatctaaacatcttctcatcaggagagagttcaatagtactcgaaccaaaagtctagtgagtctgacttctccaatccccaattttggtttgcatgtccacttacaaccatcatttctctgcaaattttccacttagtctatcaaaaatcagtgctctgaaagttctctaaaagatgcagttttttggagtctctgaatgatgacagcattctgtaaatctgcttcttccagtgtgagtgtctcatctagcaacctgaggacaggaagagctgttgccagggaaaacggaggacttctttgagatccttggtatttttcaatgaagtctttgatatggcttactctatgagtaatgttaaatttctggacaatcctttttccattggccaaccagatctgtatattagtaatgggttccaagttgttcagtggaacagcagacaaattatttttattttcaacttcaatattctttgctttagaaacaatttttggtgtggcacttcctagtctgtgaccctgtcctgaaaagggctggaacacaggcttcgtagacaaacatatttcatttttcttgtcttcaactttaacgtccacctcttctttatcaaaaattccctgtaattctgaaggtaattccccctttttgatggagttcaaaaactgctgactggcaccatcggaataacttctgaaatcgtcgttgacggtgaatccgtttttccataattttatatttacatctacctgtttcttctgttcagcgggagacacacatttggaactaaccttctgagcttcctcaaaaaggctatcaacaaaatattcacaatttgattgttgattattaccaagaggttgattatcagatcctgtttcacaaacccattcttcttttatacttttgaggttatctacgtctttcattctctttcgccttactccgggcacggcctcccggcctcggcctcactcagctcaggcaccgcaggcaccgtttggccgcgggctccgtttggctggagcccttcagagccggagcgccgccgccccagaccgcctcaggttccgcggccgcgccgctgagatcccgccagcctctctcggtcttcgccaggcgcccaagc

SEQ ID NO: 16063 - RNA, 2124 nt, Homo sapiens
  source 1..2124: mol_type = other RNA
gctgggattacaggcatgagccattgcacccggccacaattatttatatttattttactttattttatttatttttgagagggggtcttgctctgtcgccaagctggagtacagttgctcaatctcagctcactgcaacctacacttgccaggttcaagagattctcctgcctcagcctcccgagtagctgggactacagttgcgcaccgccacgcccagctaatttttgtatttttactagagatggggtttcaccatgtttgccaggatggtctcaatctgttgacctcgtgatctgcctgtctcggcctcccgaagttctgggattacaggcatgaaccactgtacccggtcgtattagctatttaaaaactcagacagctaacatttaaataaatccctgctgtctgggaatgatgtctgaatgaatattgtgaatacatatgctaatttataccatattaagattctaaacaatacagctatttaatatatcttgataactggtatttgaaaataagtctatttttctgggtagtcttttggagaaagtgcactgaatatagtttccagtcatatgctactttcttaacttgtacttatctaaacatcttctcatcaggagagagttcaatagtactcgaaccaaaagtctagtgagtctgacttctccaatccccaattttggtttgcatgtccacttacaaccatcatttctctgcaaattttccacttagtctatcaaaaatcagtgctctgaaagttctctaaaagatgcagttttttggagtctctgaatgatgacagcattctgtaaatctgcttcttccagtgtgagtgtctcatctagcaacctgaggacaggaagagctgttgccagggaaaacggaggacttctttgagatccttggtatttttcaatgaagtctttgatatggcttactctatgagtaatgttaaatttctggacaatcctttttccattggccaaccagatctgtatattagtaatgggttccaagttgttcagtggaacagcagacaaattatttttattttcaacttcaatattctttgctttagaaacaatttttggtgtggcacttcctagtctgtgaccctgtcctgaaaagggctggaacacaggcttcgtagacaaacatatttcatttttcttgtcttcaactttaacgtccacctcttctttatcaaaaattccctgtaattctgaaggtaattccccctttttgatggagttcaaaaactgctgactggcaccatcggaataacttctgaaatcgtcgttgacggtgaatccgtttttccataattttatatttacatctacctgtttcttctgttcagcgggagacacacatttggaactaaccttctgagcttcctcaaaaaggctatcaacaaaatattcacaatttgattgttgattattaccaagaggttgattatcagatcctgtttcacaaacccattcttcttttatacttttgaggttatctacgtctttcattctctttcgccttactgcctgtactcacgatgtggacaaatcccggctgccttgacttgacaggacttgagtgaagcagctctccctgggcctctctacacggtgaccgagcctcagccgcagccagcgagcagccctcctcatccaccgccaagttccagataccgcccagatgaattttttttttatcacagctgtcattctcatttctacaggcatgaaaagtgcgactcaagttcagtgtcttgcctcgggtagcttggggattcccagtcagctcctcgcgccttcgtcgccgctccccttccaccccgcgccttcgccggccgtcccctgctccatccaggccacgggggtgacggtggggtctggggcattcaggcctggctgggcatgagggcttcaggcccaattccacgcccgaactcgtcctgattagtctggcttttctggtcgccccagccctgcggtcggggagagctggaaaccaccgagctgacagcctagagcgtcgctccccggccgccgagcgctgacgccgcgccgggggcggggcagctggaggcggcagggagaggagcgagcagccgggaag

SEQ ID NO: 16064 - RNA, 1684 nt, Homo sapiens
  source 1..1684: mol_type = other RNA
gctgggattacaggcatgagccattgcacccggccacaattatttatatttattttactttattttatttatttttgagagggggtcttgctctgtcgccaagctggagtacagttgctcaatctcagctcactgcaacctacacttgccaggttcaagagattctcctgcctcagcctcccgagtagctgggactacagttgcgcaccgccacgcccagctaatttttgtatttttactagagatggggtttcaccatgtttgccaggatggtctcaatctgttgacctcgtgatctgcctgtctcggcctcccgaagttctgggattacaggcatgaaccactgtacccggtcgtattagctatttaaaaactcagacagctaacatttaaataaatccctgctgtctgggaatgatgtctgaatgaatattgtgaatacatatgctaatttataccatattaagattctaaacaatacagctatttaatatatcttgataactggtatttgaaaataagtctatttttctgggtagtcttttggagaaagtgcactgaatatagtttccagtcatatgctactttcttaacttgtacttatctaaacatcttctcatcaggagagagttcaatagtactcgaaccaaaagtctagtgagtctgacttctccaatccccaattttggtttgcatgtccacttacaaccatcatttctctgcaaattttccacttagtctatcaaaaatcagtgctctgaaagttctctaaaagatgcagttttttggagtctctgaatgatgacagcattctgtaaatctgcttcttccagtgtgagtgtctcatctagcaacctgaggacaggaagagctgttgccagggaaaacggaggacttctttgagatccttggtatttttcaatgaagtctttgatatggcttactctatgagtaatgttaaatttctggacaatcctttttccattggccaaccagatctgtatattagtaatgggttccaagttgttcagtggaacagcagacaaattatttttattttcaacttcaatattctttgctttagaaacaatttttggtgtggcacttcctagtctgtgaccctgtcctgaaaagggctggaacacaggcttcgtagacaaacatatttcatttttcttgtcttcaactttaacgtccacctcttctttatcaaaaattccctgtaattctgaaggtaattccccctttttgatggagttcaaaaactgctgactggcaccatcggaataacttctgaaatcgtcgttgacggtgaatccgtttttccataattttatatttacatctacctgtttcttctgttcagcgggagacacacatttggaactaaccttctgagcttcctcaaaaaggctatcaacaaaatattcacaatttgattgttgattattaccaagaggttgattatcagatcctgtttcacaaacccattcttcttttatacttttgaggttatctacgtctttcattctctttcgccttactgggctgggcgggaccctggctcgggctccgccgccggcgccccttcccgagtcgcaaacacgcggccctccggagcgagactccccccgacaccgacgatccgcggcggccaagccacaggccgcgacccctcggcccc

SEQ ID NO: 16065 - RNA, 1665 nt, Homo sapiens
  source 1..1665: mol_type = other RNA
gctgggattacaggcatgagccattgcacccggccacaattatttatatttattttactttattttatttatttttgagagggggtcttgctctgtcgccaagctggagtacagttgctcaatctcagctcactgcaacctacacttgccaggttcaagagattctcctgcctcagcctcccgagtagctgggactacagttgcgcaccgccacgcccagctaatttttgtatttttactagagatggggtttcaccatgtttgccaggatggtctcaatctgttgacctcgtgatctgcctgtctcggcctcccgaagttctgggattacaggcatgaaccactgtacccggtcgtattagctatttaaaaactcagacagctaacatttaaataaatccctgctgtctgggaatgatgtctgaatgaatattgtgaatacatatgctaatttataccatattaagattctaaacaatacagctatttaatatatcttgataactggtatttgaaaataagtctatttttctgggtagtcttttggagaaagtgcactgaatatagtttccagtcatatgctactttcttaacttgtacttatctaaacatcttctcatcaggagagagttcaatagtactcgaaccaaaagtctagtgagtctgacttctccaatccccaattttggtttgcatgtccacttacaaccatcatttctctgcaaattttccacttagtctatcaaaaatcagtgctctgaaagttctctaaaagatgcagttttttggagtctctgaatgatgacagcattctgtaaatctgcttcttccagtgtgagtgtctcatctagcaacctgaggacaggaagagctgttgccagggaaaacggaggacttctttgagatccttggtatttttcaatgaagtctttgatatggcttactctatgagtaatgttaaatttctggacaatcctttttccattggccaaccagatctgtatattagtaatgggttccaagttgttcagtggaacagcagacaaattatttttattttcaacttcaatattctttgctttagaaacaatttttggtgtggcacttcctagtctgtgaccctgtcctgaaaagggctggaacacaggcttcgtagacaaacatatttcatttttcttgtcttcaactttaacgtccacctcttctttatcaaaaattccctgtaattctgaaggtaattccccctttttgatggagttcaaaaactgctgactggcaccatcggaataacttctgaaatcgtcgttgacggtgaatccgtttttccataattttatatttacatctacctgtttcttctgttcagcgggagacacacatttggaactaaccttctgagcttcctcaaaaaggctatcaacaaaatattcacaatttgattgttgattattaccaagaggttgattatcagatcctgtttcacaaacccattcttcttttatacttttgaggttatctacgtctttcattctctttcgccttactgtaatcccagctactcaggaggctgaggcagaagaactgcttgaacccgggaggtggagattgtggtgagctgacatcgcgccattgcactccagcctgggcgacagggaaagactctgt

SEQ ID NO: 16066 - RNA, 2110 nt, Homo sapiens
  source 1..2110: mol_type = other RNA
gctgggattacaggcatgagccattgcacccggccacaattatttatatttattttactttattttatttatttttgagagggggtcttgctctgtcgccaagctggagtacagttgctcaatctcagctcactgcaacctacacttgccaggttcaagagattctcctgcctcagcctcccgagtagctgggactacagttgcgcaccgccacgcccagctaatttttgtatttttactagagatggggtttcaccatgtttgccaggatggtctcaatctgttgacctcgtgatctgcctgtctcggcctcccgaagttctgggattacaggcatgaaccactgtacccggtcgtattagctatttaaaaactcagacagctaacatttaaataaatccctgctgtctgggaatgatgtctgaatgaatattgtgaatacatatgctaatttataccatattaagattctaaacaatacagctatttaatatatcttgataactggtatttgaaaataagtctatttttctgggtagtcttttggagaaagtgcactgaatatagtttccagtcatatgctactttcttaacttgtacttatctaaacatcttctcatcaggagagagttcaatagtactcgaaccaaaagtctagtgagtctgacttctccaatccccaattttggtttgcatgtccacttacaaccatcatttctctgcaaattttccacttagtctatcaaaaatcagtgctctgaaagttctctaaaagatgcagttttttggagtctctgaatgatgacagcattctgtaaatctgcttcttccagtgtgagtgtctcatctagcaacctgaggacaggaagagctgttgccagggaaaacggaggacttctttgagatccttggtatttttcaatgaagtctttgatatggcttactctatgagtaatgttaaatttctggacaatcctttttccattggccaaccagatctgtatattagtaatgggttccaagttgttcagtggaacagcagacaaattatttttattttcaacttcaatattctttgctttagaaacaatttttggtgtggcacttcctagtctgtgaccctgtcctgaaaagggctggaacacaggcttcgtagacaaacatatttcatttttcttgtcttcaactttaacgtccacctcttctttatcaaaaattccctgtaattctgaaggtaattccccctttttgatggagttcaaaaactgctgactggcaccatcggaataacttctgaaatcgtcgttgacggtgaatccgtttttccataattttatatttacatctacctgtttcttctgttcagcgggagacacacatttggaactaaccttctgagcttcctcaaaaaggctatcaacaaaatattcacaatttgattgttgattattaccaagaggttgattatcagatcctgtttcacaaacccattcttcttttatacttttgaggttatctacgtctttcattctctttcgccttagatgtggacaaatcccggctgccttgacttgacaggacttgagtgaagcagctctccctgggcctctctacacggtgaccgagcctcagccgcagccagcgagcagccctcctcatccaccgccaagttccagataccgcccagatgaattttttttttatcacagctgtcattctcatttctacaggcatgaaaagtgcgactcaagttcagtgtcttgcctcgggtagcttggggattcccagtcagctcctcgcgccttcgtcgccgctccccttccaccccgcgccttcgccggccgtcccctgctccatccaggccacgggggtgacggtggggtctggggcattcaggcctggctgggcatgagggcttcaggcccaattccacgcccgaactcgtcctgattagtctggcttttctggtcgccccagccctgcggtcggggagagctggaaaccaccgagctgacagcctagagcgtcgctccccggccgccgagcgctgacgccgcgccgggggcggggcagctggaggcggcagggagaggagcgagcagccgggaag

SEQ ID NO: 16067 - RNA, 3109 nt, Homo sapiens
  source 1..3109: mol_type = other RNA
gctgggattacaggcatgagccattgcaccgggcctgttttgctgttatataaacagggcttcaatgaacatgcttggacttttctctgaacccattattagggcatatacttagaaagctaggattgtcgggcaggcacactttgaagttgactagtactgccaaactgctctctacagcgtctgaaccaattgatcctctcaccaccagcgtttgtacaagacatcctgttttaccacatccttgccaacttttgctcttgttagacttatgtttgccaatctgataggcatgaagtggcatctcatttgaagctgcattccctgcctatgaggctgagcatcttattctcattgaccatgtgggtttcctctaggcaaatcacttatgttcatatcctttgctatcctattgtagttttcggtgcaagttacaacagaaagcccaactagaaggggtttaagcaaaaaggaacgtttattagctcacgtaacaagaagtcctgggggtggttaattcagaggcctggctgtgacatcaaggaccaggttctttttgtctttttccaacaccctctcattgtgttgatttgcctcttagactggctccctcatggtcccaagatggctgccttaactctcttgtgcagacaacaacgtcagagaccgaagaaactggatgctttcttattagtctctttcccaggggtccccaccaggagaccttccagaattgcataaacgtccacacccccacttgatggaatgggagtgtctgggtggaaacggtccagggctccgtgtccagagatccagctgtgcagccatagtgccgaggcacctcggacagtccctcctcttctctcttactcctgtaatctaacgtttggccgggaatggtccctggcattccaactcatgtgtgatggatttgggcggtcagaggctcacggaacgctttgagggctgaaatccaccgataaaaaggcgggggattctgggtacatttaggtctccaggctggtatcccaaaatgtctggggggatatggaaatgtccttggaagtcggaggcttgatacagatggtgggatgggtggaggtgggatggggaagagatcattatgtccagccccctgcctccgtgcggcttctcctccccctgtagattagagcgttttctgggtcgggaaggggaggacgagatggagctcgtggccttgggttccctcctgcgtcgccccctgtaactgcgtcccccagcacgcactgctgacgcgcatccccagcccggggcggcgcgctccgcaggcatcccgcccccgactcccgctccgtcccaacatcgcgcaggcgcaagaccgggctggcgccagcgaacgcgccctctcgtggcggactggccaggtcgcagtctttgttgttgcgctggaggcggcgtacgggacaggggagaaagatgtgggtggagtctgggaggcagatgcgagaatcagatcacaatgacgagaagccctttcctttgtccctcacggcaacgtatagatgcagataaagaaaacacggcctcagacctcaagagacttagagacaggtgcacagaaactgaagctgaatgagacacactggacagcagtcattcgttcattcagcaaacattcactgggatggggagatacagggacaaaggaccagagggcttacatttaggcactggtgggcagagacggggcagaaagctggagagacggatgcggatgtcaaaaaggccaggacagagaagcgactagctcaggacagggctgggccgcaggagtgaggcggaggccggggaagtaccggcggagcctagggcacggcaagggcaccagctgtgcgaggtggggtacgagccccgacccctccagctctcctgaccgacgccccaactggggatgacaaaacggagagctaaagataggcaatgtgagcaccagaagggaccctagttgcaatggactgaagcagtcagataggtgtaaaccatgtatcatcattctactactaccaaagaagctcggactggccagagtttggaggatgctagggaaacagctctttattcagaaactgtttaatacaggaagagtccagcgtttctcccgtcttccttttacgaactttcccactcagtaaccaaatcgcaaggggcagtttctgtctataattattccagctgtctctagctggctggtcctgtccagggcttgctagacctccacgctgaagtgcttggactggggataaaggctgggtggatggcacaaacgtgacaagatcctagtcttcgaggagcttggagcagtctgtgtgattgtgttgtgcccaggaaagcacgcaggggctaaggggacacccagcttggccgggcgggccaggccgggcagccatggctgagacactcttctggactcctctcctcgtgggcaagttggggccttgttcagcggggaggcccaggatgagggggcaggatttaggggtggtaagacggaggtgtggagggcccacagaagagggatctgggttgggtgaggcaggcgccagaagggctttggggtgttaatgccatggccagctggggatccagggaatggggctgggagctgggctctgggatgaaggggctgggagctctgagggctggaggtgtcctagggcccgggtgggtctgacagcacaggcccaaagggtcgtgggccctttaatgagctggctgggccgcagcttctaagcccaggctaaatttggccctgggagggagggtggagctggcggccaggtcctctgctcctctcttggacttaggattccttttgctcagctcctactggcctctagggcaggccttcttcttccctgtattttaggggaggaaggtgggggtctccaggcccagaatggctacccttcctcctctgtaggctcctggccccgtcttcctctcctctgggctcttgggcatttagcatgggattcttttcccagtgcctttcacacatacacaccctcacacacacacacacccacacacaccctcacacacaccctcacggcaccctcacacacac

SEQ ID NO: 16068 - RNA, 3188 nt, Homo sapiens
  source 1..3188: mol_type = other RNA
gctgggattacaggcatgagccattgcaccgggcctgttttgctgttatataaacagggcttcaatgaacatgcttggacttttctctgaacccattattagggcatatacttagaaagctaggattgtcgggcaggcacactttgaagttgactagtactgccaaactgctctctacagcgtctgaaccaattgatcctctcaccaccagcgtttgtacaagacatcctgttttaccacatccttgccaacttttgctcttgttagacttatgtttgccaatctgataggcatgaagtggcatctcatttgaagctgcattccctgcctatgaggctgagcatcttattctcattgaccatgtgggtttcctctaggcaaatcacttatgttcatatcctttgctatcctattgtagttttcggtgcaagttacaacagaaagcccaactagaaggggtttaagcaaaaaggaacgtttattagctcacgtaacaagaagtcctgggggtggttaattcagaggcctggctgtgacatcaaggaccaggttctttttgtctttttccaacaccctctcattgtgttgatttgcctcttagactggctccctcatggtcccaagatggctgccttaactctcttgtgcagacaacaacgtcagagaccgaagaaactggatgctttcttattagtctctttcccaggggtccccaccaggagaccttccagaattgcataaacgtccacacccccacttgatggaatgggagtgtctgggtggaaacggtccagggctccgtgtccagagatccagctgtgcagccatagtgccgaggcacctcggacagtccctcctcttctctcttactcctgtaatctaacgtttggccgggaatggtccctggcattccaactcatgtgtgatggatttgggcggtcagaggctcacggaacgctttgagggctgaaatccaccgataaaaaggcgggggattctgggtacatttaggtctccaggctggtatcccaaaatgtctggggggatatggaaatgtccttggaagtcggaggcttgatacagatggtgggatgggtggaggtgggatggggaagagatcattatgtccagccccctgcctccgtgcggcttctcctccccctgtagattagagcgttttctgggtcgggaaggggaggacgagatggagctcgtggccttgggttccctcctgcgtcgccccctgtaactgcgtcccccagcacgcactgctgacgcgcatccccagcccggggcggcgcgctccgcaggcatcccgcccccgactcccgctccgtcccaacatcgcgcaggcgcaagaccgggctggcgccagcgaacgcgccctctcgtggcggactggccaggtcgcagtctttgttgttgcgctggaggcggcgtacgggacaggggagaaagatgtgggtggagtctgggaggcagatgcgagaatcagatcacaatgacgagaagccctttcctttgtccctcacggcaacgtatagatgcagataaagaaaacacggcctcagacctcaagagacttagagacaggtgcacagaaactgaagctgaatgagacacactggacagcagtcattcgttcattcagcaaacattcactgggatggggagatacagggacaaaggaccagagggcttacatttaggcactggtgggcagagacggggcagaaagctggagagacggatgcggatgtcaaaaaggccaggacagagaagcgactagctcaggacagggctgggccgcaggagtgaggcggaggccggggaagtaccggcggagcctagggcacggcaagggcaccagctgtgcgaggtggggtacgagccccgacccctccagctctcctgaccgacgccccaactggggatgacaaaacggagagctaaagataggcaatgtgagcaccagaagggaccctagttgcaatggactgaagcagtcagataggtgtaaaccatgtatcatcattctactactaccaaagaagctcggactggccagagtttggaggatgctagggaaacagctctttattcagaaactgtttaatacaggaagagtccagcgtttctcccgtcttccttttacgaactttcccactcagtaaccaaatcgcaaggggcagtttctgtctataattattccagctgtctctagctggctggtcctgtccagggcttgctagacctccacgctgaagtgcttggactggggataaaggctgggtggatggcacctacgtttgctgttaaggaagctgccgccagccagctacacctactagttaccaggccctgtgccaggcccaaggatacaaacgtgacaagatcctagtcttcgaggagcttggagcagtctgtgtgattgtgttgtgcccaggaaagcacgcaggggctaaggggacacccagcttggccgggcgggccaggccgggcagccatggctgagacactcttctggactcctctcctcgtgggcaagttggggccttgttcagcggggaggcccaggatgagggggcaggatttaggggtggtaagacggaggtgtggagggcccacagaagagggatctgggttgggtgaggcaggcgccagaagggctttggggtgttaatgccatggccagctggggatccagggaatggggctgggagctgggctctgggatgaaggggctgggagctctgagggctggaggtgtcctagggcccgggtgggtctgacagcacaggcccaaagggtcgtgggccctttaatgagctggctgggccgcagcttctaagcccaggctaaatttggccctgggagggagggtggagctggcggccaggtcctctgctcctctcttggacttaggattccttttgctcagctcctactggcctctagggcaggccttcttcttccctgtattttaggggaggaaggtgggggtctccaggcccagaatggctacccttcctcctctgtaggctcctggccccgtcttcctctcctctgggctcttgggcatttagcatgggattcttttcccagtgcctttcacacatacacaccctcacacacacacacacccacacacaccctcacacacaccctcacggcaccctcacacacac

SEQ ID NO: 16069 - RNA, 2011 nt, Homo sapiens
  source 1..2011: mol_type = other RNA
gctgggattacaggcatgagccattgcaccgggcctgttttgctgttatataaacagggcttcaatgaacatgcttggacttttctctgaacccattattagggcatatacttagaaagctaggattgtcgggcaggcacactttgaagttgactagtactgccaaactgctctctacagcgtctgaaccaattgatcctctcaccaccagcgtttgtacaagacatcctgttttaccacatccttgccaacttttgctcttgttagacttatgtttgccaatctgataggcatgaagtggcatctcatttgaagctgcattccctgcctatgaggctgagcatcttattctcattgaccatgtgggtttcctctaggcaaatcacttatgttcatatcctttgctatcctattgtagttttcggtgcaagttacaacagaaagcccaactagaaggggtttaagcaaaaaggaacgtttattagctcacgtaacaagaagtcctgggggtggttaattcagaggcctggctgtgacatcaaggaccaggttctttttgtctttttccaacaccctctcattgtgttgatttgcctcttagactggctccctcatggtcccaagatggctgccttaactctcttgtgcagacaacaacgtcagagaccgaagaaactggatgctttcttattagtctctttcccaggggtccccaccaggagaccttccagaattgcataaacgtccacacccccacttgatggaatgggagtgtctgggtggaaacggtccagggctccgtgtccagagatccagctgtgcagccatagtgccgaggcacctcggacagtccctcctcttctctcttactcctgtaatctaacgtttggccgggaatggtccctggcattccaactcatgtgtgatggatttgggcggtcagaggctcacggaacgctttgagggctgaaatccaccgataaaaaggcgggggattctgggtacatttaggtctccaggctggtatcccaaaatgtctgtctctagctggctggtcctgtccagggcttgctagacctccacgctgaagtgcttggactggggataaaggctgggtggatggcacctacgtttgctgttaaggaagctgccgccagccagctacacctactagttaccaggccctgtgccaggcccaaggatacaaacgtgacaagatcctagtcttcgaggagcttggagcagtctgtgtgattgtgttgtgcccaggaaagcacgcaggggctaaggggacacccagcttggccgggcgggccaggccgggcagccatggctgagacactcttctggactcctctcctcgtgggcaagttggggccttgttcagcggggaggcccaggatgagggggcaggatttaggggtggtaagacggaggtgtggagggcccacagaagagggatctgggttgggtgaggcaggcgccagaagggctttggggtgttaatgccatggccagctggggatccagggaatggggctgggagctgggctctgggatgaaggggctgggagctctgagggctggaggtgtcctagggcccgggtgggtctgacagcacaggcccaaagggtcgtgggccctttaatgagctggctgggccgcagcttctaagcccaggctaaatttggccctgggagggagggtggagctggcggccaggtcctctgctcctctcttggacttaggattccttttgctcagctcctactggcctctagggcaggccttcttcttccctgtattttaggggaggaaggtgggggtctccaggcccagaatggctacccttcctcctctgtaggctcctggccccgtcttcctctcctctgggctcttgggcatttagcatgggattcttttcccagtgcctttcacacatacacaccctcacacacacacacacccacacacaccctcacacacaccctcacggcaccctcacacacac

SEQ ID NO: 16070 - RNA, 1853 nt, Homo sapiens
  source 1..1853: mol_type = other RNA
gctgggattacaggcatgagccattgcaccgggcctgttttgctgttatataaacagggcttcaatgaacatgcttggacttttctctgaacccattattagggcatatacttagaaagctaggattgtcgggcaggcacactttgaagttgactagtactgccaaactgctctctacagcgtctgaaccaattgatcctctcaccaccagcgtttgtacaagacatcctgttttaccacatccttgccaacttttgctcttgttagacttatgtttgccaatctgataggcatgaagtggcatctcatttgaagctgcattccctgcctatgaggctgagcatcttattctcattgaccatgtgggtttcctctaggcaaatcacttatgttcatatcctttgctatcctattgtagttttcggtgcaagttacaacagaaagcccaactagaaggggtttaagcaaaaaggaacgtttattagctcacgtaacaagaagtcctgggggtggttaattcagaggcctggctgtgacatcaaggaccaggttctttttgtctttttccaacaccctctcattgtgttgatttgcctcttagactggctccctcatggtcccaagatggctgccttaactctcttgtgcagacaacaacgtcagagaccgaagaaactggatgctttcttattagtctctttcccaggggtccccaccaggagaccttccagaattgcataaacgtccacacccccacttgatggaatgggagtgtctgggtggaaacggtccagggctccgtgtccagagatccagctgtgcagccatagtgccgaggcacctcggacagtccctcctcttctctcttactcctgtaatctgtctctagctggctggtcctgtccagggcttgctagacctccacgctgaagtgcttggactggggataaaggctgggtggatggcacctacgtttgctgttaaggaagctgccgccagccagctacacctactagttaccaggccctgtgccaggcccaaggatacaaacgtgacaagatcctagtcttcgaggagcttggagcagtctgtgtgattgtgttgtgcccaggaaagcacgcaggggctaaggggacacccagcttggccgggcgggccaggccgggcagccatggctgagacactcttctggactcctctcctcgtgggcaagttggggccttgttcagcggggaggcccaggatgagggggcaggatttaggggtggtaagacggaggtgtggagggcccacagaagagggatctgggttgggtgaggcaggcgccagaagggctttggggtgttaatgccatggccagctggggatccagggaatggggctgggagctgggctctgggatgaaggggctgggagctctgagggctggaggtgtcctagggcccgggtgggtctgacagcacaggcccaaagggtcgtgggccctttaatgagctggctgggccgcagcttctaagcccaggctaaatttggccctgggagggagggtggagctggcggccaggtcctctgctcctctcttggacttaggattccttttgctcagctcctactggcctctagggcaggccttcttcttccctgtattttaggggaggaaggtgggggtctccaggcccagaatggctacccttcctcctctgtaggctcctggccccgtcttcctctcctctgggctcttgggcatttagcatgggattcttttcccagtgcctttcacacatacacaccctcacacacacacacacccacacacaccctcacacacaccctcacggcaccctcacacacac

SEQ ID NO: 16071 - RNA, 4457 nt, Homo sapiens
  source 1..4457: mol_type = other RNA
gctgggattacaggcatgagccattgcacctggccaaagtagtggaactgagcctgtttcctccacaggccacaccaccctgcaaagagttgcccccaccccaagcccctagctatatcccaggcctggaaataactagtgtcaggagaaaaaacgtccaaagccttcctgtgtggccgttgctgctctcctcaccacccctcactaggaccgagtggcttcccagcttccatcaaggccagccacgatcttgcaaccaattgtgggcaacctcaattcagatgcctagagagctcctcttctcagtcccctgagccacaggcccctggccagcctctccctgagcagtcgttttctttgcagcttcctccgtcactgctcaactctcggttatttttctcaccctaccttagaactcatgaaatcccccttgctttgcccacctacatgcatatcattctcagctctgtatctccaacccaaatacccagtgcttatttggagtctcaaaatcacgtagtccacaaatgagcccaggtgccctcttgtatctctcctccctcccctgtatccagtcaccacttcccaacacagccctctaagcatctctccattctggccatccacttctcccctctccattctggccacccacctcccatcttagttcaggccttcctttctcacctggaccacggtcacagcccccttcatggccactagtggagggcagactgaaagggacagctgctaagacagggaagtggcaatggtaacagcagagtttatgggcacctcacaacctgaaggtggtgagacggcagtaagctgggatgaggatgtgggcactgctgcacagagatcaacaaatgcagagagaaggcagtgtctcggggctggagctcagaggtaaggggtggttgaagtgttccctggaaatcagtcaaggtgatgctaatgactgcttggggagacccaggactgaggctgaggacagccacagctaactgtcagcagagaatgaaccagaacattagtagcctgggtggcaggacaggcaagagggctctgctgagtgagaactgagatgaggctgtgaaatgaatgccagattcggtggcatgggattcactggtggcctatcaagaaccctgctgtgagccgggcgcaggggctcacacctgtattcccagcactttgggaggccaaggcaggcggatcacctggggtctggagttcgagaccagcctggccatcatggtgaaaccccatctctactaaaaatataaaaattagccagccatggtggcacatgcctgtagtctcagctacgcaggaggctaaggcaggagaattgcttgagcctggaaggcagaggttgcagtgagctgagatcgccccactgcactccacctgggtgacacagcgagactgtctcaaaaaccctgctgtggagtgacagggtttactgagcacaaggtggaacatgagggaatggactagtttctctagagtagggggagggcccacggaggaggaagctcaaagcgaggcagaaggggacatcaacagcgtcttcccaactcaggcaccagagacagacagtcccgggtttgagtccagctctactcttttccagctgagtgaccctgggcagccttactcatccgttcagtttccttttctgttaaattgtgggaacagcaagggctgcatggtgacccacgtcgagcagtggacaacctcctgaacgcagcacagcagaggcagcaggaccacaaaacaggggcctcagaggggcaggccctggcctcggtctccatgggaagtgagcaagttcacaggagttggcccagggagcagcaccctgtggtacaagcaggaggatggtggtgccatctttggtgcctgggtactggaggagggtgaggccaccaacagcgctgctggcagcagaggagggcagaggaactcaggatcagggcgtcagaggtagtataggccaggagcctgcaaacagcagcagcagggaagagggtcaccaatcactctccaggggacaaaattaccctccacgcagcagccatcctgctctgcacccacacaaggtcccaatgcagcagcacccatatttcctaagtgccaaggcccatgtgcagaggtggccacgcctagtggaacagcccacagcccacatatcagttccccttgccccagctggaacacgggtgtctctgctgcctccatgcggctggcaccctgcccatccctccctgaccacagccttaaacggaggggagcagggaggctgcagagccttggggttttccctcctggtccaaggctgctttgtacaggcccatccttgccttcaacagcaatatgggcaccacttaagacctcagatataaaaggtgcattctctccttgggaaaggcttttgaaattattctgcaaagcagaaagaaaagcttcagcccctaccaagagcacctgcagcctggcactctcctcaggcagtcttctgagactcacctcccaagtgccacagtgccctgaaggaccccccactccccatgagttctttgacagacacttcagttcttccttttctacttagcctgaaagaaaaaccagattctccctgatcccctgagggggtgtcaattctagtggccctgctgactcatgttagtcctccagattgtgctgcttctgccagtgtacccacttgcatcagaacagtccgcccactacccaaggaaattctgccaagaaaagaagccctgtctctccagacattcattcccaggatttagtgtaaagtaacgtggaactgcccttccaaaaactgcttgttaagtttcaggtacacaattaacctgcccaattaattttgcagaaccttgaaataaaacatgttttacagtaagttcacacacaggcttaatgcaaaccagagtaatgcacagatgattgccaagaccatattgacaaattgtgattagattataacgcatagtagcctgccttacattcagcaagttcaaacaggacacaaaaccagtcaactgaacacagagcagctctcttcagaagcacttccaatgagtgatgcagagatttcaaaaatacaaagcaggcaacttatatacagcaaatcctcacactgcctggacatgtgccacttttttgttgtttttaatatatttttccttcctggttgctaatttagactgaattcttaaggatttatcttgatgacttagaaaaatacacctgtcctttctcactttgtttcaggtagtacagtcatgaaattgagtaagtctcttaaaaaaatgaaagtccacagatcccattgtggaaggtttcaggaacccctccccaggtaatgatcacgggatcttcaacagctcaaggagtgctccaacagctccaaaataaccctcgtgttccgaaaaaagtgctttcaactgccccttggaccaataatccaaagcatatgccaaaagccgcatggcgatcgtattaattctcaagaaatttccaacaaataccacctggttaatgttttcattaagggcacacattcttgctattgagccaatgttgttggtgatggtgatcaaagtcgctctggccaggtcctctttactgacagcctctcgcttctccttgctcatcatgtttccaaagcttgaagccacagcccagcctggcagtccaaacctctcatagtcccctccataaatatctcgtactagtttatccactttggtgctatctccacgagatgccatttcaagagcttcttcaaaagtggtacagccagtaagaagacagcagagaccaaaaaaagttcctcctccaagactagtacctgtgacccgtttgtaattatctttggaatatactgctaagatgctaacccctgagccaatgttcaccagaagcagaggatacggatttttcaaatcaaatggtaacttctgacacttttcagaatcagcagggttttcaaagtaatagcactgtgaccgtccattgaatccgactgagtcaatgtataaaattcctttgatcaagcaatctagttcatccagtttgcaaagctgaagatcacctatctttgcgtccacacagagtcaggtccttcagctcgaggtgcacgtcccgaatgcctgtagacccataagccacattggaggtcaggtacttccgaatgcttttaagactttccacttcttcctcttcttcttcagcagtgatgtctttgggttcaaaatataccagcttgaccagagttccaccgatatccagtccaaaccatggaaaaacaatgggtgcgggggggcccccgaaggtaccgctttcggagcacccgaggcctccagccggatgtcaggccacgcaccaacgagggaccaccgtgcggggacagtgtccgcgcgcgg

SEQ ID NO: 16072 - RNA, 4682 nt, Homo sapiens
  source 1..4682: mol_type = other RNA
gctgggattacaggcatgagccattgcacctggccaaagtagtggaactgagcctgtttcctccacaggccacaccaccctgcaaagagttgcccccaccccaagcccctagctatatcccaggcctggaaataactagtgtcaggagaaaaaacgtccaaagccttcctgtgtggccgttgctgctctcctcaccacccctcactaggaccgagtggcttcccagcttccatcaaggccagccacgatcttgcaaccaattgtgggcaacctcaattcagatgcctagagagctcctcttctcagtcccctgagccacaggcccctggccagcctctccctgagcagtcgttttctttgcagcttcctccgtcactgctcaactctcggttatttttctcaccctaccttagaactcatgaaatcccccttgctttgcccacctacatgcatatcattctcagctctgtatctccaacccaaatacccagtgcttatttggagtctcaaaatcacgtagtccacaaatgagcccaggtgccctcttgtatctctcctccctcccctgtatccagtcaccacttcccaacacagccctctaagcatctctccattctggccatccacttctcccctctccattctggccacccacctcccatcttagttcaggccttcctttctcacctggaccacggtcacagcccccttcatggccactagtggagggcagactgaaagggacagctgctaagacagggaagtggcaatggtaacagcagagtttatgggcacctcacaacctgaaggtggtgagacggcagtaagctgggatgaggatgtgggcactgctgcacagagatcaacaaatgcagagagaaggcagtgtctcggggctggagctcagaggtaaggggtggttgaagtgttccctggaaatcagtcaaggtgatgctaatgactgcttggggagacccaggactgaggctgaggacagccacagctaactgtcagcagagaatgaaccagaacattagtagcctgggtggcaggacaggcaagagggctctgctgagtgagaactgagatgaggctgtgaaatgaatgccagattcggtggcatgggattcactggtggcctatcaagaaccctgctgtgagccgggcgcaggggctcacacctgtattcccagcactttgggaggccaaggcaggcggatcacctggggtctggagttcgagaccagcctggccatcatggtgaaaccccatctctactaaaaatataaaaattagccagccatggtggcacatgcctgtagtctcagctacgcaggaggctaaggcaggagaattgcttgagcctggaaggcagaggttgcagtgagctgagatcgccccactgcactccacctgggtgacacagcgagactgtctcaaaaaccctgctgtggagtgacagggtttactgagcacaaggtggaacatgagggaatggactagtttctctagagtagggggagggcccacggaggaggaagctcaaagcgaggcagaaggggacatcaacagcgtcttcccaactcaggcaccagagacagacagtcccgggtttgagtccagctctactcttttccagctgagtgaccctgggcagccttactcatccgttcagtttccttttctgttaaattgtgggaacagcaagggctgcatggtgacccacgtcgagcagtggacaacctcctgaacgcagcacagcagaggcagcaggaccacaaaacaggggcctcagaggggcaggccctggcctcggtctccatgggaagtgagcaagttcacaggagttggcccagggagcagcaccctgtggtacaagcaggaggatggtggtgccatctttggtgcctgggtactggaggagggtgaggccaccaacagcgctgctggcagcagaggagggcagaggaactcaggatcagggcgtcagaggtagtataggccaggagcctgcaaacagcagcagcagggaagagggtcaccaatcactctccaggggacaaaattaccctccacgcagcagccatcctgctctgcacccacacaaggtcccaatgcagcagcacccatatttcctaagtgccaaggcccatgtgcagaggtggccacgcctagtggaacagcccacagcccacatatcagttccccttgccccagctggaacacgggtgtctctgctgcctccatgcggctggcaccctgcccatccctccctgaccacagccttaaacggaggggagcagggaggctgcagagccttggggttttccctcctggtccaaggctgctttgtacaggcccatccttgccttcaacagcaatatgggcaccacttaagacctcagatataaaaggtgcattctctccttgggaaaggcttttgaaattattctgcaaagcagaaagaaaagcttcagcccctaccaagagcacctgcagcctggcactctcctcaggcagtcttctgagactcacctcccaagtgccacagtgccctgaaggaccccccactccccatgagttctttgacagacacttcagttcttccttttctacttagcctgaaagaaaaaccagattctccctgatcccctgagggggtgtcaattctagtggccctgctgactcatgttagtcctccagattgtgctgcttctgccagtgtacccacttgcatcagaacagtccgcccactacccaaggaaattctgccaagaaaagaagccctgtctctccagacattcattcccaggatttagtgtaaagtaacgtggaactgcccttccaaaaactgcttgttaagtttcaggtacacaattaacctgcccaattaattttgcagaaccttgaaataaaacatgttttacagtaagttcacacacaggcttaatgcaaaccagagtaatgcacagatgattgccaagaccatattgacaaattgtgattagattataacgcatagtagcctgccttacattcagcaagttcaaacaggacacaaaaccagtcaactgaacacagagcagctctcttcagaagcacttccaatgagtgatgcagagatttcaaaaatacaaagcaggcaacttatatacagcaaatcctcacactgcctggacatgtgccacttttttgttgtttttaatatatttttccttcctggttgctaatttagactgaattcttaaggatttatcttgatgacttagaaaaatacacctgtcctttctcactttgtttcaggtagtacagtcatgaaattgagtaagtctcttaaaaaaatgaaagtccacagatcccattgtggaaggtttcaggaacccctccccaggtaatgatcacgggatcttcaacagctcaaggagtgctccaacagctccaaaataaccctcgtgttccgaaaaaagtgctttcaactgccccttggaccaataatccaaagcatatgccaaaagccgcatggcgatcgtattaattctcaagaaatttccaacaaataccacctggttaatgttttcattaagggcacacattcttgctattgagccaatgttgttggtgatggtgatcaaagtcgctctggccaggtcctctttactgacagcctctcgcttctccttgctcatcatgtttccaaagcttgaagccacagcccagcctggcagtccaaacctctcatagtcccctccataaatatctcgtactagtttatccactttggtgctatctccacgagatgccatttcaagagcttcttcaaaagtggtacagccagtaagaagacagcagagaccaaaaaaagttcctcctccaagactagtacctgtgacccgtttgtaattatctttggaatatactgctaagatgctaacccctgagccaatgttcaccagaagcagaggatacggatttttcaaatcaaatggtaacttctgacacttttcagaatcagcagggttttcaaagtaatagcactgtgaccgtccattgaatccgactgagtcaatgtataaaattcctttgatcaagcaatctagttcatccagtttgcaaagctgaagatcacctatctttgcgtccacacagagtcaggtccttcagctcgaggtgcacgtcccgaatgcctgtagacccataagccacattggaggtcaggtacttccgaatgcttttaagactttccacttcttcctcttcttcttcagcagtgatgtctttgggttcaaaatataccagcttgaccagagttccaccgatatccagtccaaaccatggaaaaagcggccgctttttcctcaggctttcgacgcgctggcgggagaccgaggtggggccgctgtaagagcccagtcgatcccgcctcgtgccctcagccgaggccccgaccgcgggcaccgacgcgctgctcgcccggcgccgcagtggctcctgccgccgcccttcggggtccccggccgcctgctccccagccgacgagacggaggtggcggaagccctgccgtggcgctccatgggcgcgccgagccggccccctcccatccgcagcagcagtcgctgccgcccgagcaagccccccagcgtcggattccttctcgcctcctccgcggcagtccagccagagc

SEQ ID NO: 16073 - RNA, 4600 nt, Homo sapiens
  source 1..4600: mol_type = other RNA
gctgggattacaggcatgagccattgcacctggccaaagtagtggaactgagcctgtttcctccacaggccacaccaccctgcaaagagttgcccccaccccaagcccctagctatatcccaggcctggaaataactagtgtcaggagaaaaaacgtccaaagccttcctgtgtggccgttgctgctctcctcaccacccctcactaggaccgagtggcttcccagcttccatcaaggccagccacgatcttgcaaccaattgtgggcaacctcaattcagatgcctagagagctcctcttctcagtcccctgagccacaggcccctggccagcctctccctgagcagtcgttttctttgcagcttcctccgtcactgctcaactctcggttatttttctcaccctaccttagaactcatgaaatcccccttgctttgcccacctacatgcatatcattctcagctctgtatctccaacccaaatacccagtgcttatttggagtctcaaaatcacgtagtccacaaatgagcccaggtgccctcttgtatctctcctccctcccctgtatccagtcaccacttcccaacacagccctctaagcatctctccattctggccatccacttctcccctctccattctggccacccacctcccatcttagttcaggccttcctttctcacctggaccacggtcacagcccccttcatggccactagtggagggcagactgaaagggacagctgctaagacagggaagtggcaatggtaacagcagagtttatgggcacctcacaacctgaaggtggtgagacggcagtaagctgggatgaggatgtgggcactgctgcacagagatcaacaaatgcagagagaaggcagtgtctcggggctggagctcagaggtaaggggtggttgaagtgttccctggaaatcagtcaaggtgatgctaatgactgcttggggagacccaggactgaggctgaggacagccacagctaactgtcagcagagaatgaaccagaacattagtagcctgggtggcaggacaggcaagagggctctgctgagtgagaactgagatgaggctgtgaaatgaatgccagattcggtggcatgggattcactggtggcctatcaagaaccctgctgtgagccgggcgcaggggctcacacctgtattcccagcactttgggaggccaaggcaggcggatcacctggggtctggagttcgagaccagcctggccatcatggtgaaaccccatctctactaaaaatataaaaattagccagccatggtggcacatgcctgtagtctcagctacgcaggaggctaaggcaggagaattgcttgagcctggaaggcagaggttgcagtgagctgagatcgccccactgcactccacctgggtgacacagcgagactgtctcaaaaaccctgctgtggagtgacagggtttactgagcacaaggtggaacatgagggaatggactagtttctctagagtagggggagggcccacggaggaggaagctcaaagcgaggcagaaggggacatcaacagcgtcttcccaactcaggcaccagagacagacagtcccgggtttgagtccagctctactcttttccagctgagtgaccctgggcagccttactcatccgttcagtttccttttctgttaaattgtgggaacagcaagggctgcatggtgacccacgtcgagcagtggacaacctcctgaacgcagcacagcagaggcagcaggaccacaaaacaggggcctcagaggggcaggccctggcctcggtctccatgggaagtgagcaagttcacaggagttggcccagggagcagcaccctgtggtacaagcaggaggatggtggtgccatctttggtgcctgggtactggaggagggtgaggccaccaacagcgctgctggcagcagaggagggcagaggaactcaggatcagggcgtcagaggtagtataggccaggagcctgcaaacagcagcagcagggaagagggtcaccaatcactctccaggggacaaaattaccctccacgcagcagccatcctgctctgcacccacacaaggtcccaatgcagcagcacccatatttcctaagtgccaaggcccatgtgcagaggtggccacgcctagtggaacagcccacagcccacatatcagttccccttgccccagctggaacacgggtgtctctgctgcctccatgcggctggcaccctgcccatccctccctgaccacagccttaaacggaggggagcagggaggctgcagagccttggggttttccctcctggtccaaggctgctttgtacaggcccatccttgccttcaacagcaatatgggcaccacttaagacctcagatataaaaggtgcattctctccttgggaaaggcttttgaaattattctgcaaagcagaaagaaaagcttcagcccctaccaagagcacctgcagcctggcactctcctcaggcagtcttctgagactcacctcccaagtgccacagtgccctgaaggaccccccactccccatgagttctttgacagacacttcagttcttccttttctacttagcctgaaagaaaaaccagattctccctgatcccctgagggggtgtcaattctagtggccctgctgactcatgttagtcctccagattgtgctgcttctgccagtgtacccacttgcatcagaacagtccgcccactacccaaggaaattctgccaagaaaagaagccctgtctctccagacattcattcccaggatttagtgtaaagtaacgtggaactgcccttccaaaaactgcttgttaagtttcaggtacacaattaacctgcccaattaattttgcagaaccttgaaataaaacatgttttacagtaagttcacacacaggcttaatgcaaaccagagtaatgcacagatgattgccaagaccatattgacaaattgtgattagattataacgcatagtagcctgccttacattcagcaagttcaaacaggacacaaaaccagtcaactgaacacagagcagctctcttcagaagcacttccaatgagtgatgcagagatttcaaaaatacaaagcaggcaacttatatacagcaaatcctcacactgcctggacatgtgccacttttttgttgtttttaatatatttttccttcctggttgctaatttagactgaattcttaaggatttatcttgatgacttagaaaaatacacctgtcctttctcactttgtttcaggtagtacagtcatgaaattgagtaagtctcttaaaaaaatgaaagtccacagatcccattgtggaaggtttcaggaacccctccccaggtaatgatcacgggatcttcaacagctcaaggagtgctccaacagctccaaaataaccctcgtgttccgaaaaaagtgctttcaactgccccttggaccaataatccaaagcatatgccaaaagccgcatggcgatcgtattaattctcaagaaatttccaacaaataccacctggttaatgttttcattaagggcacacattcttgctattgagccaatgttgttggtgatggtgatcaaagtcgctctggccaggtcctctttactgacagcctctcgcttctccttgctcatcatgtttccaaagcttgaagccacagcccagcctggcagtccaaacctctcatagtcccctccataaatatctcgtactagtttatccactttggtgctatctccacgagatgccatttcaagagcttcttcaaaagtggtacagccagtaagaagacagcagagaccaaaaaaagttcctcctccaagactagtacctgtgacccgtttgtaattatctttggaatatactgctaagatgctaacccctgagccaatgttcaccagaagcagaggatacggatttttcaaatcaaatggtaacttctgacacttttcagaatcagcagggttttcaaagtaatagcactgtgaccgtccattgaatccgactgagtcaatgtataaaattcctttgatcaagcaatctagttcatccagtttgcaaagctgaagatcacctattgtgagaaaatcctgctcaaatttgtacgctccacctccagtggcacaaaagacagtgtggagactcgagaagtttttatctctgcccatttgaataaaagcaggcatgtcatgagtgggaaagcgtataaagtgcagattgcctttgcgtccacacagagtcaggtccttcagctcgaggtgcacgtcccgaatgcctgtagacccataagccacattggaggtcaggtacttccgaatgcttttaagactttccacttcttcctcttcttcttcagcagtgatgtctttgggttcaaaatataccagcttgaccagagttccaccgatatccagtccaaaccatggaaaaacaatgggtgcgggggggcccccgaaggtaccgctttcggagcacccgaggcctccagccggatgtcaggccacgcaccaacgagggaccaccgtgcggggacagtgtccgcgcgcgg

SEQ ID NO: 16074 - RNA, 4993 nt, Homo sapiens
  source 1..4993: mol_type = other RNA
gctgggattacaggcatgagccattgcacctggccaaagtagtggaactgagcctgtttcctccacaggccacaccaccctgcaaagagttgcccccaccccaagcccctagctatatcccaggcctggaaataactagtgtcaggagaaaaaacgtccaaagccttcctgtgtggccgttgctgctctcctcaccacccctcactaggaccgagtggcttcccagcttccatcaaggccagccacgatcttgcaaccaattgtgggcaacctcaattcagatgcctagagagctcctcttctcagtcccctgagccacaggcccctggccagcctctccctgagcagtcgttttctttgcagcttcctccgtcactgctcaactctcggttatttttctcaccctaccttagaactcatgaaatcccccttgctttgcccacctacatgcatatcattctcagctctgtatctccaacccaaatacccagtgcttatttggagtctcaaaatcacgtagtccacaaatgagcccaggtgccctcttgtatctctcctccctcccctgtatccagtcaccacttcccaacacagccctctaagcatctctccattctggccatccacttctcccctctccattctggccacccacctcccatcttagttcaggccttcctttctcacctggaccacggtcacagcccccttcatggccactagtggagggcagactgaaagggacagctgctaagacagggaagtggcaatggtaacagcagagtttatgggcacctcacaacctgaaggtggtgagacggcagtaagctgggatgaggatgtgggcactgctgcacagagatcaacaaatgcagagagaaggcagtgtctcggggctggagctcagaggtaaggggtggttgaagtgttccctggaaatcagtcaaggtgatgctaatgactgcttggggagacccaggactgaggctgaggacagccacagctaactgtcagcagagaatgaaccagaacattagtagcctgggtggcaggacaggcaagagggctctgctgagtgagaactgagatgaggctgtgaaatgaatgccagattcggtggcatgggattcactggtggcctatcaagaaccctgctgtgagccgggcgcaggggctcacacctgtattcccagcactttgggaggccaaggcaggcggatcacctggggtctggagttcgagaccagcctggccatcatggtgaaaccccatctctactaaaaatataaaaattagccagccatggtggcacatgcctgtagtctcagctacgcaggaggctaaggcaggagaattgcttgagcctggaaggcagaggttgcagtgagctgagatcgccccactgcactccacctgggtgacacagcgagactgtctcaaaaaccctgctgtggagtgacagggtttactgagcacaaggtggaacatgagggaatggactagtttctctagagtagggggagggcccacggaggaggaagctcaaagcgaggcagaaggggacatcaacagcgtcttcccaactcaggcaccagagacagacagtcccgggtttgagtccagctctactcttttccagctgagtgaccctgggcagccttactcatccgttcagtttccttttctgttaaattgtgggaacagcaagggctgcatggtgacccacgtcgagcagtggacaacctcctgaacgcagcacagcagaggcagcaggaccacaaaacaggggcctcagaggggcaggccctggcctcggtctccatgggaagtgagcaagttcacaggagttggcccagggagcagcaccctgtggtacaagcaggaggatggtggtgccatctttggtgcctgggtactggaggagggtgaggccaccaacagcgctgctggcagcagaggagggcagaggaactcaggatcagggcgtcagaggtagtataggccaggagcctgcaaacagcagcagcagggaagagggtcaccaatcactctccaggggacaaaattaccctccacgcagcagccatcctgctctgcacccacacaaggtcccaatgcagcagcacccatatttcctaagtgccaaggcccatgtgcagaggtggccacgcctagtggaacagcccacagcccacatatcagttccccttgccccagctggaacacgggtgtctctgctgcctccatgcggctggcaccctgcccatccctccctgaccacagccttaaacggaggggagcagggaggctgcagagccttggggttttccctcctggtccaaggctgctttgtacaggcccatccttgccttcaacagcaatatgggcaccacttaagacctcagatataaaaggtgcattctctccttgggaaaggcttttgaaattattctgcaaagcagaaagaaaagcttcagcccctaccaagagcacctgcagcctggcactctcctcaggcagtcttctgagactcacctcccaagtgccacagtgccctgaaggaccccccactccccatgagttctttgacagacacttcagttcttccttttctacttagcctgaaagaaaaaccagattctccctgatcccctgagggggtgtcaattctagtggccctgctgactcatgttagtcctccagattgtgctgcttctgccagtgtacccacttgcatcagaacagtccgcccactacccaaggaaattctgccaagaaaagaagccctgtctctccagacattcattcccaggatttagtgtaaagtaacgtggaactgcccttccaaaaactgcttgttaagtttcaggtacacaattaacctgcccaattaattttgcagaaccttgaaataaaacatgttttacagtaagttcacacacaggcttaatgcaaaccagagtaatgcacagatgattgccaagaccatattgacaaattgtgattagattataacgcatagtagcctgccttacattcagcaagttcaaacaggacacaaaaccagtcaactgaacacagagcagctctcttcagaagcacttccaatgagtgatgcagagatttcaaaaatacaaagcaggcaacttatatacagcaaatcctcacactgcctggacatgtgccacttttttgttgtttttaatatatttttccttcctggttgctaatttagactgaattcttaaggatttatcttgatgacttagaaaaatacacctgtcctttctcactttgtttcaggtagtacagtcatgaaattgagtaagtctcttaaaaaaatgaaagtccacagatcccattgtggaaggtttcaggaacccctccccaggtaatgatcacgggatcttcaacagctcaaggagtgctccaacagctccaaaataaccctcgtgttccgaaaaaagtgctttcaactgccccttggaccaataatccaaagcatatgccaaaagccgcatggcgatcgtattaattctcaagaaatttccaacaaataccacctggttaatgttttcattaagggcacacattcttgctattgagccaatgttgttggtgatggtgatcaaagtcgctctggccaggtcctctttactgacagcctctcgcttctccttgctcatcatgtttccaaagcttgaagccacagcccagcctggcagtccaaacctctcatagtcccctccataaatatctcgtactagtttatccactttggtgctatctccacgagatgccatttcaagagcttcttcaaaagtggtacagccagtaagaagacagcagagaccaaaaaaagttcctcctccaagactagtacctgtgacccgtttgtaattatctttggaatatactgctaagatgctaacccctgagccaatgttcaccagaagcagaggatacggatttttcaaatcaaatggtaacttctgacacttttcagaatcagcagggttttcaaagtaatagcactgtgaccgtccattgaatccgactgagtcaatgtataaaattcctttgatcaagcaatctagttcatccagtttgcaaagctgaagatcacctattgtgagaaaatcctgctcaaatttgtacgctccacctccagtggcacaaaagacagtgtggagactcgagaagtttttatctctgcccatttgaataaaagcaggcatgtcatgagtgggaaagcgtataaagtgcagattgcctttgcgtccacacagagtcaggtccttcagctcgaggtgcacgtcccgaatgcctgtagacccataagccacattggaggtcaggtacttccgaatgcttttaagactttccacttcttcctcttcttcttcagcagtgatgtctttgggttcaaaatataccagcttgaccagagttccaccgatatccagtccaaaccatggaaaaactcagagccacgaggctaatgagttaccaaagctcttagtagacgactgccaggtcgggcacaatggctcccgtctatatcccagcactttgggaggccgaagtgggaagatcgcttgagaccaggaggaattcaagaccagcctgggcaacataagagatcccatctgcggccgctttttcctcaggctttcgacgcgctggcgggagaccgaggtggggccgctgtaagagcccagtcgatcccgcctcgtgccctcagccgaggccccgaccgcgggcaccgacgcgctgctcgcccggcgccgcagtggctcctgccgccgcccttcggggtccccggccgcctgctccccagccgacgagacggaggtggcggaagccctgccgtggcgctccatgggcgcgccgagccggccccctcccatccgcagcagcagtcgctgccgcccgagcaagccccccagcgtcggattccttctcgcctcctccgcggcagtccagccagagc

SEQ ID NO: 16075 - RNA, 4607 nt, Homo sapiens
  source 1..4607: mol_type = other RNA
gctgggattacaggcatgagccattgcacctggccaaagtagtggaactgagcctgtttcctccacaggccacaccaccctgcaaagagttgcccccaccccaagcccctagctatatcccaggcctggaaataactagtgtcaggagaaaaaacgtccaaagccttcctgtgtggccgttgctgctctcctcaccacccctcactaggaccgagtggcttcccagcttccatcaaggccagccacgatcttgcaaccaattgtgggcaacctcaattcagatgcctagagagctcctcttctcagtcccctgagccacaggcccctggccagcctctccctgagcagtcgttttctttgcagcttcctccgtcactgctcaactctcggttatttttctcaccctaccttagaactcatgaaatcccccttgctttgcccacctacatgcatatcattctcagctctgtatctccaacccaaatacccagtgcttatttggagtctcaaaatcacgtagtccacaaatgagcccaggtgccctcttgtatctctcctccctcccctgtatccagtcaccacttcccaacacagccctctaagcatctctccattctggccatccacttctcccctctccattctggccacccacctcccatcttagttcaggccttcctttctcacctggaccacggtcacagcccccttcatggccactagtggagggcagactgaaagggacagctgctaagacagggaagtggcaatggtaacagcagagtttatgggcacctcacaacctgaaggtggtgagacggcagtaagctgggatgaggatgtgggcactgctgcacagagatcaacaaatgcagagagaaggcagtgtctcggggctggagctcagaggtaaggggtggttgaagtgttccctggaaatcagtcaaggtgatgctaatgactgcttggggagacccaggactgaggctgaggacagccacagctaactgtcagcagagaatgaaccagaacattagtagcctgggtggcaggacaggcaagagggctctgctgagtgagaactgagatgaggctgtgaaatgaatgccagattcggtggcatgggattcactggtggcctatcaagaaccctgctgtgagccgggcgcaggggctcacacctgtattcccagcactttgggaggccaaggcaggcggatcacctggggtctggagttcgagaccagcctggccatcatggtgaaaccccatctctactaaaaatataaaaattagccagccatggtggcacatgcctgtagtctcagctacgcaggaggctaaggcaggagaattgcttgagcctggaaggcagaggttgcagtgagctgagatcgccccactgcactccacctgggtgacacagcgagactgtctcaaaaaccctgctgtggagtgacagggtttactgagcacaaggtggaacatgagggaatggactagtttctctagagtagggggagggcccacggaggaggaagctcaaagcgaggcagaaggggacatcaacagcgtcttcccaactcaggcaccagagacagacagtcccgggtttgagtccagctctactcttttccagctgagtgaccctgggcagccttactcatccgttcagtttccttttctgttaaattgtgggaacagcaagggctgcatggtgacccacgtcgagcagtggacaacctcctgaacgcagcacagcagaggcagcaggaccacaaaacaggggcctcagaggggcaggccctggcctcggtctccatgggaagtgagcaagttcacaggagttggcccagggagcagcaccctgtggtacaagcaggaggatggtggtgccatctttggtgcctgggtactggaggagggtgaggccaccaacagcgctgctggcagcagaggagggcagaggaactcaggatcagggcgtcagaggtagtataggccaggagcctgcaaacagcagcagcagggaagagggtcaccaatcactctccaggggacaaaattaccctccacgcagcagccatcctgctctgcacccacacaaggtcccaatgcagcagcacccatatttcctaagtgccaaggcccatgtgcagaggtggccacgcctagtggaacagcccacagcccacatatcagttccccttgccccagctggaacacgggtgtctctgctgcctccatgcggctggcaccctgcccatccctccctgaccacagccttaaacggaggggagcagggaggctgcagagccttggggttttccctcctggtccaaggctgctttgtacaggcccatccttgccttcaacagcaatatgggcaccacttaagacctcagatataaaaggtgcattctctccttgggaaaggcttttgaaattattctgcaaagcagaaagaaaagcttcagcccctaccaagagcacctgcagcctggcactctcctcaggcagtcttctgagactcacctcccaagtgccacagtgccctgaaggaccccccactccccatgagttctttgacagacacttcagttcttccttttctacttagcctgaaagaaaaaccagattctccctgatcccctgagggggtgtcaattctagtggccctgctgactcatgttagtcctccagattgtgctgcttctgccagtgtacccacttgcatcagaacagtccgcccactacccaaggaaattctgccaagaaaagaagccctgtctctccagacattcattcccaggatttagtgtaaagtaacgtggaactgcccttccaaaaactgcttgttaagtttcaggtacacaattaacctgcccaattaattttgcagaaccttgaaataaaacatgttttacagtaagttcacacacaggcttaatgcaaaccagagtaatgcacagatgattgccaagaccatattgacaaattgtgattagattataacgcatagtagcctgccttacattcagcaagttcaaacaggacacaaaaccagtcaactgaacacagagcagctctcttcagaagcacttccaatgagtgatgcagagatttcaaaaatacaaagcaggcaacttatatacagcaaatcctcacactgcctggacatgtgccacttttttgttgtttttaatatatttttccttcctggttgctaatttagactgaattcttaaggatttatcttgatgacttagaaaaatacacctgtcctttctcactttgtttcaggtagtacagtcatgaaattgagtaagtctcttaaaaaaatgaaagtccacagatcccattgtggaaggtttcaggaacccctccccaggtaatgatcacgggatcttcaacagctcaaggagtgctccaacagctccaaaataaccctcgtgttccgaaaaaagtgctttcaactgccccttggaccaataatccaaagcatatgccaaaagccgcatggcgatcgtattaattctcaagaaatttccaacaaataccacctggttaatgttttcattaagggcacacattcttgctattgagccaatgttgttggtgatggtgatcaaagtcgctctggccaggtcctctttactgacagcctctcgcttctccttgctcatcatgtttccaaagcttgaagccacagcccagcctggcagtccaaacctctcatagtcccctccataaatatctcgtactagtttatccactttggtgctatctccacgagatgccatttcaagagcttcttcaaaagtggtacagccagtaagaagacagcagagaccaaaaaaagttcctcctccaagactagtacctgtgacccgtttgtaattatctttggaatatactgctaagatgctaacccctgagccaatgttcaccagaagcagaggatacggatttttcaaatcaaatggtaacttctgacacttttcagaatcagcagggttttcaaagtaatagcactgtgaccgtccattgaatccgactgagtcaatgtataaaattcctttgatcaagcaatctagttcatccagtttgcaaagctgaagatcacctattgtgagaaaatcctgctcaaatttgtacgctccacctccagtggcacaaaagacagtgtggagactcgagaagtttttatctctgcccatttgaataaaagcaggcatgtcatgagtgggaaagcgtataaagtgcagattgcctttgcgtccacacagagtcaggtccttcagctcgaggtgcacgtcccgaatgcctgtagacccataagccacattggaggtcaggtacttccgaatgcttttaagactttccacttcttcctcttcttcttcagcagtgatgtctttgggttcaaaatataccagcttgaccagagttccaccgatatccagtccaaaccatggaaaaacttagcctttgtccctcggcctagttccgcagctgccgtcgaggccgccagcccctcccccagcatgtttgggctaagccgcctcctttccgcctgcgttggagagagaggtaccagaaggaat

SEQ ID NO: 16076 - RNA, 4825 nt, Homo sapiens
  source 1..4825: mol_type = other RNA
gctgggattacaggcatgagccattgcacctggccaaagtagtggaactgagcctgtttcctccacaggccacaccaccctgcaaagagttgcccccaccccaagcccctagctatatcccaggcctggaaataactagtgtcaggagaaaaaacgtccaaagccttcctgtgtggccgttgctgctctcctcaccacccctcactaggaccgagtggcttcccagcttccatcaaggccagccacgatcttgcaaccaattgtgggcaacctcaattcagatgcctagagagctcctcttctcagtcccctgagccacaggcccctggccagcctctccctgagcagtcgttttctttgcagcttcctccgtcactgctcaactctcggttatttttctcaccctaccttagaactcatgaaatcccccttgctttgcccacctacatgcatatcattctcagctctgtatctccaacccaaatacccagtgcttatttggagtctcaaaatcacgtagtccacaaatgagcccaggtgccctcttgtatctctcctccctcccctgtatccagtcaccacttcccaacacagccctctaagcatctctccattctggccatccacttctcccctctccattctggccacccacctcccatcttagttcaggccttcctttctcacctggaccacggtcacagcccccttcatggccactagtggagggcagactgaaagggacagctgctaagacagggaagtggcaatggtaacagcagagtttatgggcacctcacaacctgaaggtggtgagacggcagtaagctgggatgaggatgtgggcactgctgcacagagatcaacaaatgcagagagaaggcagtgtctcggggctggagctcagaggtaaggggtggttgaagtgttccctggaaatcagtcaaggtgatgctaatgactgcttggggagacccaggactgaggctgaggacagccacagctaactgtcagcagagaatgaaccagaacattagtagcctgggtggcaggacaggcaagagggctctgctgagtgagaactgagatgaggctgtgaaatgaatgccagattcggtggcatgggattcactggtggcctatcaagaaccctgctgtgagccgggcgcaggggctcacacctgtattcccagcactttgggaggccaaggcaggcggatcacctggggtctggagttcgagaccagcctggccatcatggtgaaaccccatctctactaaaaatataaaaattagccagccatggtggcacatgcctgtagtctcagctacgcaggaggctaaggcaggagaattgcttgagcctggaaggcagaggttgcagtgagctgagatcgccccactgcactccacctgggtgacacagcgagactgtctcaaaaaccctgctgtggagtgacagggtttactgagcacaaggtggaacatgagggaatggactagtttctctagagtagggggagggcccacggaggaggaagctcaaagcgaggcagaaggggacatcaacagcgtcttcccaactcaggcaccagagacagacagtcccgggtttgagtccagctctactcttttccagctgagtgaccctgggcagccttactcatccgttcagtttccttttctgttaaattgtgggaacagcaagggctgcatggtgacccacgtcgagcagtggacaacctcctgaacgcagcacagcagaggcagcaggaccacaaaacaggggcctcagaggggcaggccctggcctcggtctccatgggaagtgagcaagttcacaggagttggcccagggagcagcaccctgtggtacaagcaggaggatggtggtgccatctttggtgcctgggtactggaggagggtgaggccaccaacagcgctgctggcagcagaggagggcagaggaactcaggatcagggcgtcagaggtagtataggccaggagcctgcaaacagcagcagcagggaagagggtcaccaatcactctccaggggacaaaattaccctccacgcagcagccatcctgctctgcacccacacaaggtcccaatgcagcagcacccatatttcctaagtgccaaggcccatgtgcagaggtggccacgcctagtggaacagcccacagcccacatatcagttccccttgccccagctggaacacgggtgtctctgctgcctccatgcggctggcaccctgcccatccctccctgaccacagccttaaacggaggggagcagggaggctgcagagccttggggttttccctcctggtccaaggctgctttgtacaggcccatccttgccttcaacagcaatatgggcaccacttaagacctcagatataaaaggtgcattctctccttgggaaaggcttttgaaattattctgcaaagcagaaagaaaagcttcagcccctaccaagagcacctgcagcctggcactctcctcaggcagtcttctgagactcacctcccaagtgccacagtgccctgaaggaccccccactccccatgagttctttgacagacacttcagttcttccttttctacttagcctgaaagaaaaaccagattctccctgatcccctgagggggtgtcaattctagtggccctgctgactcatgttagtcctccagattgtgctgcttctgccagtgtacccacttgcatcagaacagtccgcccactacccaaggaaattctgccaagaaaagaagccctgtctctccagacattcattcccaggatttagtgtaaagtaacgtggaactgcccttccaaaaactgcttgttaagtttcaggtacacaattaacctgcccaattaattttgcagaaccttgaaataaaacatgttttacagtaagttcacacacaggcttaatgcaaaccagagtaatgcacagatgattgccaagaccatattgacaaattgtgattagattataacgcatagtagcctgccttacattcagcaagttcaaacaggacacaaaaccagtcaactgaacacagagcagctctcttcagaagcacttccaatgagtgatgcagagatttcaaaaatacaaagcaggcaacttatatacagcaaatcctcacactgcctggacatgtgccacttttttgttgtttttaatatatttttccttcctggttgctaatttagactgaattcttaaggatttatcttgatgacttagaaaaatacacctgtcctttctcactttgtttcaggtagtacagtcatgaaattgagtaagtctcttaaaaaaatgaaagtccacagatcccattgtggaaggtttcaggaacccctccccaggtaatgatcacgggatcttcaacagctcaaggagtgctccaacagctccaaaataaccctcgtgttccgaaaaaagtgctttcaactgccccttggaccaataatccaaagcatatgccaaaagccgcatggcgatcgtattaattctcaagaaatttccaacaaataccacctggttaatgttttcattaagggcacacattcttgctattgagccaatgttgttggtgatggtgatcaaagtcgctctggccaggtcctctttactgacagcctctcgcttctccttgctcatcatgtttccaaagcttgaagccacagcccagcctggcagtccaaacctctcatagtcccctccataaatatctcgtactagtttatccactttggtgctatctccacgagatgccatttcaagagcttcttcaaaagtggtacagccagtaagaagacagcagagaccaaaaaaagttcctcctccaagactagtacctgtgacccgtttgtaattatctttggaatatactgctaagatgctaacccctgagccaatgttcaccagaagcagaggatacggatttttcaaatcaaatggtaacttctgacacttttcagaatcagcagggttttcaaagtaatagcactgtgaccgtccattgaatccgactgagtcaatgtataaaattcctttgatcaagcaatctagttcatccagtttgcaaagctgaagatcacctattgtgagaaaatcctgctcaaatttgtacgctccacctccagtggcacaaaagacagtgtggagactcgagaagtttttatctctgcccatttgaataaaagcaggcatgtcatgagtgggaaagcgtataaagtgcagattgcctttgcgtccacacagagtcaggtccttcagctcgaggtgcacgtcccgaatgcctgtagacccataagccacattggaggtcaggtacttccgaatgcttttaagactttccacttcttcctcttcttcttcagcagtgatgtctttgggttcaaaatataccagcttgaccagagttccaccgatatccagtccaaaccatggaaaaagcggccgctttttcctcaggctttcgacgcgctggcgggagaccgaggtggggccgctgtaagagcccagtcgatcccgcctcgtgccctcagccgaggccccgaccgcgggcaccgacgcgctgctcgcccggcgccgcagtggctcctgccgccgcccttcggggtccccggccgcctgctccccagccgacgagacggaggtggcggaagccctgccgtggcgctccatgggcgcgccgagccggccccctcccatccgcagcagcagtcgctgccgcccgagcaagccccccagcgtcggattccttctcgcctcctccgcggcagtccagccagagc

SEQ ID NO: 16077 - RNA, 5289 nt, Homo sapiens
  source 1..5289: mol_type = other RNA
gctgggattacaggcatgagccattgcacctggccaaagtagtggaactgagcctgtttcctccacaggccacaccaccctgcaaagagttgcccccaccccaagcccctagctatatcccaggcctggaaataactagtgtcaggagaaaaaacgtccaaagccttcctgtgtggccgttgctgctctcctcaccacccctcactaggaccgagtggcttcccagcttccatcaaggccagccacgatcttgcaaccaattgtgggcaacctcaattcagatgcctagagagctcctcttctcagtcccctgagccacaggcccctggccagcctctccctgagcagtcgttttctttgcagcttcctccgtcactgctcaactctcggttatttttctcaccctaccttagaactcatgaaatcccccttgctttgcccacctacatgcatatcattctcagctctgtatctccaacccaaatacccagtgcttatttggagtctcaaaatcacgtagtccacaaatgagcccaggtgccctcttgtatctctcctccctcccctgtatccagtcaccacttcccaacacagccctctaagcatctctccattctggccatccacttctcccctctccattctggccacccacctcccatcttagttcaggccttcctttctcacctggaccacggtcacagcccccttcatggccactagtggagggcagactgaaagggacagctgctaagacagggaagtggcaatggtaacagcagagtttatgggcacctcacaacctgaaggtggtgagacggcagtaagctgggatgaggatgtgggcactgctgcacagagatcaacaaatgcagagagaaggcagtgtctcggggctggagctcagaggtaaggggtggttgaagtgttccctggaaatcagtcaaggtgatgctaatgactgcttggggagacccaggactgaggctgaggacagccacagctaactgtcagcagagaatgaaccagaacattagtagcctgggtggcaggacaggcaagagggctctgctgagtgagaactgagatgaggctgtgaaatgaatgccagattcggtggcatgggattcactggtggcctatcaagaaccctgctgtgagccgggcgcaggggctcacacctgtattcccagcactttgggaggccaaggcaggcggatcacctggggtctggagttcgagaccagcctggccatcatggtgaaaccccatctctactaaaaatataaaaattagccagccatggtggcacatgcctgtagtctcagctacgcaggaggctaaggcaggagaattgcttgagcctggaaggcagaggttgcagtgagctgagatcgccccactgcactccacctgggtgacacagcgagactgtctcaaaaaccctgctgtggagtgacagggtttactgagcacaaggtggaacatgagggaatggactagtttctctagagtagggggagggcccacggaggaggaagctcaaagcgaggcagaaggggacatcaacagcgtcttcccaactcaggcaccagagacagacagtcccgggtttgagtccagctctactcttttccagctgagtgaccctgggcagccttactcatccgttcagtttccttttctgttaaattgtgggaacagcaagggctgcatggtgacccacgtcgagcagtggacaacctcctgaacgcagcacagcagaggcagcaggaccacaaaacaggggcctcagaggggcaggccctggcctcggtctccatgggaagtgagcaagttcacaggagttggcccagggagcagcaccctgtggtacaagcaggaggatggtggtgccatctttggtgcctgggtactggaggagggtgaggccaccaacagcgctgctggcagcagaggagggcagaggaactcaggatcagggcgtcagaggtagtataggccaggagcctgcaaacagcagcagcagggaagagggtcaccaatcactctccaggggacaaaattaccctccacgcagcagccatcctgctctgcacccacacaaggtcccaatgcagcagcacccatatttcctaagtgccaaggcccatgtgcagaggtggccacgcctagtggaacagcccacagcccacatatcagttccccttgccccagctggaacacgggtgtctctgctgcctccatgcggctggcaccctgcccatccctccctgaccacagccttaaacggaggggagcagggaggctgcagagccttggggttttccctcctggtccaaggctgctttgtacaggcccatccttgccttcaacagcaatatgggcaccacttaagacctcagatataaaaggtgcattctctccttgggaaaggcttttgaaattattctgcaaagcagaaagaaaagcttcagcccctaccaagagcacctgcagcctggcactctcctcaggcagtcttctgagactcacctcccaagtgccacagtgccctgaaggaccccccactccccatgagttctttgacagacacttcagttcttccttttctacttagcctgaaagaaaaaccagattctccctgatcccctgagggggtgtcaattctagtggccctgctgactcatgttagtcctccagattgtgctgcttctgccagtgtacccacttgcatcagaacagtccgcccactacccaaggaaattctgccaagaaaagaagccctgtctctccagacattcattcccaggatttagtgtaaagtaacgtggaactgcccttccaaaaactgcttgttaagtttcaggtacacaattaacctgcccaattaattttgcagaaccttgaaataaaacatgttttacagtaagttcacacacaggcttaatgcaaaccagagtaatgcacagatgattgccaagaccatattgacaaattgtgattagattataacgcatagtagcctgccttacattcagcaagttcaaacaggacacaaaaccagtcaactgaacacagagcagctctcttcagaagcacttccaatgagtgatgcagagatttcaaaaatacaaagcaggcaacttatatacagcaaatcctcacactgcctggacatgtgccacttttttgttgtttttaatatatttttccttcctggttgctaatttagactgaattcttaaggatttatcttgatgacttagaaaaatacacctgtcctttctcactttgtttcaggtagtacagtcatgaaattgagtaagtctcttaaaaaaatgaaagtccacagatcccattgtggaaggtttcaggaacccctccccaggtaatgatcacgggatcttcaacagctcaaggagtgctccaacagctccaaaataaccctcgtgttccgaaaaaagtgctttcaactgccccttggaccaataatccaaagcatatgccaaaagccgcatggcgatcgtattaattctcaagaaatttccaacaaataccacctggttaatgttttcattaagggcacacattcttgctattgagccaatgttgttggtgatggtgatcaaagtcgctctggccaggtcctctttactgacagcctctcgcttctccttgctcatcatgtttccaaagcttgaagccacagcccagcctggcagtccaaacctctcatagtcccctccataaatatctcgtactagtttatccactttggtgctatctccacgagatgccatttcaagagcttcttcaaaagtggtacagccagtaagaagacagcagagaccaaaaaaagttcctcctccaagactagtacctgtgacccgtttgtaattatctttggaatatactgctaagatgctaacccctgagccaatgttcaccagaagcagaggatacggatttttcaaatcaaatggtaacttctgacacttttcagaatcagcagggttttcaaagtaatagcactgtgaccgtccattgaatccgactgagtcaatgtataaaattcctttgatcaagcaatctagttcatccagtttgcaaagctgaagatcacctattgtgagaaaatcctgctcaaatttgtacgctccacctccagtggcacaaaagacagtgtggagactcgagaagtttttatctctgcccatttgaataaaagcaggcatgtcatgagtgggaaagcgtataaagtgcagattgcctttgcgtccacacagagtcaggtccttcagctcgaggtgcacgtcccgaatgcctgtagacccataagccacattggaggtcaggtacttccgaatgcttttaagactttccacttcttcctcttcttcttcagcagtgatgtctttgggttcaaaatataccagcttgaccagagttccaccgatatccagtccaaaccatggaaaaagcggccgctttttcctcaggctttcgacgcgctggcgggagaccgaggtggggccgctgtaagagcccagtcgatcccgcctcgtgccctcagccgaggccccgaccgcgggcaccgacgcgctgctcgcccggcgccgcagtggctcctgccgccgcccttcggggtccccggccgcctgctccccagccgacgagacggaggtggcggaagccctgccgtggcgctccatgggcgcgccgagccggccccctcccatccgcagcagcagtcgctgccgcccgagcaagccccccagcgtcggattccttctcgcctcctccgcggcagtccagccagagcagaggcgcgccctcggccggccgcctcttccgttgcgccaacgcgcaggaagccaatccgacgaggctggggacggcccaaaggcctcgcgtccagtcggctccctaactcgaggaggattgaccgtgcctccgtccaatgagaggctatcgtgacggggcggggagagggtggtggaggaggggatccgggttccgcggaggaagagaaggcggtgtagcccagaagagagtgatggcggcgccgcccaatggacgcgtgggtggaagggcccgagcctcctcatccaccccctccttccgccccccacttgtgcatgcctctgcccccccgggccgcggaactctcctggggcgaccccgagtcccaccccgctgctccgtgccgtcctcgcagctcgagccctcctccagcccagcagtgctcccgcagcgtctggccgctggtcgtcggcagacgaaagg

SEQ ID NO: 16078 - RNA, 952 nt, Homo sapiens
  source 1..952: mol_type = other RNA
gctgggattacaggcatgagccattgcacctggccaaggaaacatatttcctaacagagtaatagaaattactgtaaatggtcacaatatcactagaactgaattttgtccctttcaaaaatatgtcagaataataaagagaatatagaaaacaatcatttttttcaaagttttttaattgttaccaatgccattttactactttttatctttttcatgcagtttcagaagaaattagcaatatctaactctcttttcatagtcatagtgatttcaagagtttcagtctctgggatatagaatgctttggcactggtacattccaccagctcaggaagagttatcaacagcttcttctgaggagtacgaaggtcaaggattgtttcctggatatcaatttgaatatcagaagggtttgtatttggcaatttaattttagccactagttcactgcaacaacctgttgaggagtccttttttgacaaccctaaaaatatatcttcagttcccacctgctgtctgaatataatctcatactctgggatttctctaacatcccacatatcatcatattctgctccttctggaatctcttctgaattccagatgtcctcattattttcctcgctggtttcagggatgactttgagctcttctatttggggtggtccaatattcccaggacccatggctccaatagtagataaaccatttgtctgtccatagtcagaatcatcctcttcttcaggattaagtagcttagagagggcttccagagctgtaactgaagaaacactctcaaagtctacattttgagattccatattttctgtcttcatattttcagaatccatattttcagattccattatcttggtcagttttcccgtctctggctaggctccgaaaatagactgtgcagagcgtggcgtctctccgttgctagggtaac

SEQ ID NO: 16079 - RNA, 1227 nt, Homo sapiens
  source 1..1227: mol_type = other RNA
gctgggattacaggcatgagccattgcacctggccaaggaaacatatttcctaacagagtaatagaaattactgtaaatggtcacaatatcactagaactgaattttgtccctttcaaaaatatgtcagaataataaagagaatatagaaaacaatcatttttttcaaagttttttaattgttaccaatgccattttactactttttatctttttcatgcagtttcagaagaaattagcaatatctaactctcttttcatagtcatagtgatttcaagagtttcagtctctgggatatagaatgctttggcactggtacattccaccagctcaggaagagttatcaacagcttcttctgaggagtacgaaggtcaaggattgtttcctggatatcaatttgaatatcagaagggtttgtatttggcaatttaattttagccactagttcactgcaacaacctgttgaggagtccttttttgacaaccctaaaaatatatcttcagttcccacctgctgtctgaatataatctcatactctgggatttctctaacatcccacatatcatcatattctgctccttctggaatctcttctgaattccagatgtcctcattattttcctcgctggtttcagggatgactttgagctcttctatttggggtggtccaatattcccaggacccatggctccaatagtagataaaccatttgtctgtccatagtcagaatcatcctcttcttcaggattaagtagcttagagagggcttccagagctgtaactgaagaaacactctcaaagtctacattttgagattccatattttctgtcttcatattttcagaatccatattttcagattccattattctcccaatcagcccttggcgagtagcaggtcttgtaggtacaagtagtctctgcacagtacactcgggcccaccaagtgaaggtctgattacttctcactcctcagcttatctaaccaagcaacactggaaccctcagaccacagcgttcaagttgtcgcacaaaggacattattcacgtagtaagtactggggccatttttttttcagtctgaagtgtgatatcccccaaaacatttcctaaccaaggcatgctaggccaggataaatcgtgccttggtcagttttcccgtctctggctaggctccgaaaatagactgtgcagagcgtggcgtctctccgttgctagggtaac

SEQ ID NO: 16080 - RNA, 3793 nt, Homo sapiens
  source 1..3793: mol_type = other RNA
gctgggattacaggcatgagccattgcacctggccacttacccattttaaagtgtacaaatgcattggtattaaatgtattcacaatattgtgcaaacaccaggtctctccagcttccaaactttctcatcaccctgtaaaaaacatcttgtatccagcaagcagtcactccccattcctccctccccatgccctggtaacctctaatctgctttctatccctatagatttgcttcttctgaatatatcatgtaaaaagaatcataccataggtgaccttccctgcctggcatctttcatttgcataatgcttctaaggaccatctatgttatagcatgtaccagcacttcattcctttctacagctgaatcatatcccacagtatgtgcataccacggtttgcagtttgtttatccattcatacattggattgtttgcactttttggctttattttattatttttagagacgaggtctcactctgtcatccaggctggagtgcagtggcaccaccatggttcgttgcagcctcaacctccttgagctcaaaggatcctcctgcctcagccacacaagtagctgggacgaccggtatgcactaccacgcctggctgatttttaaatttttgtagggatggggtcccactatgttgcccaggctgttctcaaactcctggcttcaagcaatcctcccgcctcagcctcccaaagtgctgggattacaactgtgagccactgtgcccaggtccatgttgagctttttgaggaagtgccagactgtggttgggatcattctttcctctagatacccaaagctggtacctccttgtcattcagggctcagctcccatatcacctccccagaccaccccagctcaaacagtgctcctctcccaagtcactctcttgtctgctgccatcttttcaccatctggagtttattacccagtaggatgtaggtgatctcggacctcttagtctccactgtgacccacaacctagcacagtttctggtagacggaggttctcaataaatgcttactgaatgactgatctcaggtagtcaaaggtaaagagctgtaataatgtgaggcactgtcactgtcaccttaggtcgctgttaggacctccccctgggtgactcatctgtttgtttgtttatttatttatttatttatttatttatttatttatttattttagatggagtctcactctgtcgtccaggctggagttcagaggcacaatctcggctcactgccacctctgcctcccgggttcaagtgattctcctgcctcagcctccccaccacacctggctaatttttgtgtttttagtagagatgagttttcaccatgttggccaggctggtctccaactcctgacctcaagtggtccgcctgcctcggcctcccaaagtgctgggattacaggcatgagccaccacgcccagccaactcacctgtttaaatggtcaacttcctcctctctgaggaaagaataaaaaccaggaaagagaaaccattggcgatgcttctttctcagccctttcctgttagtgactcagcacaggtatctccttcactatccccagctcctgaggtgcaacaagcagcccttagtgacaactgaatggttatcattgtcatcatcatcaatccatctcggttctgatatctgcaggctggtcattcagatcagatactcgctctcggcatccaaagcgctggtggcttcatccaggatgaggactggggggttccgcaccagagcccgggccatggccacccgctgcttctggccacctgacagctgggcgcccttctcccctgtctctgtgctgtagccgtcctggagttccatgatgaagccgtgggcattggccttctgtgcggcctccaccaccatctcgaaaggcacagtgggcaggccgtaggagatgttatccgtgatggagcgggcgaacagcacgggctcctggctcaccagggagatcacacggtgcaagtacttgtggtcgtaggcgctgatgggcttgccgtccagcagcacccggcccccctccagggggtagaagttctccaggatgttgacacaggagctcttcccactgcccgagggccccaccagggccgtcaccttgccgggggacaggctgaaggagacattctccatacaatctcccaggacaaactcgtagatgatgaaggcgatgaggttgccgctggtcatctggcctgagatgacaaggtggcccccgtagtagaggatgctgacctggaccaccagcagtgtgagcccgctgccccagacgtagtacatgtaggcagctgcctccttcctgttcagcttgtacacctgctgcagcttccgcaggtacacctctgcctcctcctcctcattggcgaagctccggacagtcttcatggcactgatggtctcctccgccgtgttgctcgctctggccagggcattctggacctctttggagagcctcttgtagtacttgccgtagatgttggacaccatcatgatgatggggaagcccatgaaggtgaccaaggagagctgccatgagaggctgaacatgaagaccaccacgcccgtgaccttgactgtgttccgcaggaagacattgatgttctgggagaccaggtcgctgaccatggtggtgtccgaggtcaggcgggagatgaggtcccctgtgcggttctcatcaaagaagcttgtctcctgggacaccagtgagcggaagagacagtttcgaaggcgaatgttcagtctggcaaatatgagggtaaaaatgccgccccgaatacctgccaatggccagcaggcacacgatgacgacagccgtgctgaactgatccatgcttttctggatgacgatgccatcaatggcgcggcccgtgtagtagggcaggaaggtctctcccagagctgccacgatgaggaagaaggaggcggccacgaggaaggccacgtcgggcttggtgtaggagagcagcttctgcagcgtggccccagacgcctgctcgggcggtggccggccgctcccagggaagccctcagcctcggtggccgcccctggctccagggcctgggtgcctggccgcacggtggacagcagccaccagagcaggaaggatgcgccgagtgaaatgtacgtccacacgaacagggcccaaaaccaggggtcccggatgggcctgcgcacctctgagaagagcagcagcttcaccatggcatagatgcccacgaagaggcacacgagggtgatgaccagccacgaggcccgcagccgccggggccccagcgcactgttcttggccacaccaatggtggctcccagcagcaggcagctgcggtacaggcaggctgcccagagatccagcaccgagtcaaagatgttgaagtggcggatgtcctccaggaggctgcggtccaggtggctgaagacatagatggccgtggtcacgcagatgtccacactcatgaaggccaaagtcaccaccaccgccttccacagccgcatcctgctggttggaggtgggcgggtgctgaaggccaggttgtagctcacgggggcaaggccatcatcatccacagggcgaggccaggcctgttacctggcaccaggtgagctctgggagggggcgcgcagcaggctcgggtctggggtgcagtttccgcgctgctcattgaagactgcgccggacgcggtcctcgctccgctcttcccgctgctcctccccgcctcccacccgcgctgcgccgctgcaaggtcgga

SEQ ID NO: 16081 - RNA, 3816 nt, Homo sapiens
  source 1..3816: mol_type = other RNA
gctgggattacaggcatgagccattgcacctggccacttacccattttaaagtgtacaaatgcattggtattaaatgtattcacaatattgtgcaaacaccaggtctctccagcttccaaactttctcatcaccctgtaaaaaacatcttgtatccagcaagcagtcactccccattcctccctccccatgccctggtaacctctaatctgctttctatccctatagatttgcttcttctgaatatatcatgtaaaaagaatcataccataggtgaccttccctgcctggcatctttcatttgcataatgcttctaaggaccatctatgttatagcatgtaccagcacttcattcctttctacagctgaatcatatcccacagtatgtgcataccacggtttgcagtttgtttatccattcatacattggattgtttgcactttttggctttattttattatttttagagacgaggtctcactctgtcatccaggctggagtgcagtggcaccaccatggttcgttgcagcctcaacctccttgagctcaaaggatcctcctgcctcagccacacaagtagctgggacgaccggtatgcactaccacgcctggctgatttttaaatttttgtagggatggggtcccactatgttgcccaggctgttctcaaactcctggcttcaagcaatcctcccgcctcagcctcccaaagtgctgggattacaactgtgagccactgtgcccaggtccatgttgagctttttgaggaagtgccagactgtggttgggatcattctttcctctagatacccaaagctggtacctccttgtcattcagggctcagctcccatatcacctccccagaccaccccagctcaaacagtgctcctctcccaagtcactctcttgtctgctgccatcttttcaccatctggagtttattacccagtaggatgtaggtgatctcggacctcttagtctccactgtgacccacaacctagcacagtttctggtagacggaggttctcaataaatgcttactgaatgactgatctcaggtagtcaaaggtaaagagctgtaataatgtgaggcactgtcactgtcaccttaggtcgctgttaggacctccccctgggtgactcatctgtttgtttgtttatttatttatttatttatttatttatttatttatttattttagatggagtctcactctgtcgtccaggctggagttcagaggcacaatctcggctcactgccacctctgcctcccgggttcaagtgattctcctgcctcagcctccccaccacacctggctaatttttgtgtttttagtagagatgagttttcaccatgttggccaggctggtctccaactcctgacctcaagtggtccgcctgcctcggcctcccaaagtgctgggattacaggcatgagccaccacgcccagccaactcacctgtttaaatggtcaacttcctcctctctgaggaaagaataaaaaccaggaaagagaaaccattggcgatgcttctttctcagccctttcctgttagtgactcagcacaggtatctccttcactatccccagctcctgaggtgcaacaagcagcccttagtgacaactgaatggttatcattgtcatcatcatcaatccatctcggttctgatatctgcaggctggtcattcagatcagatactcgctctcggcatccaaagcgctggtggcttcatccaggatgaggactggggggttccgcaccagagcccgggccatggccacccgctgcttctggccacctgacagctgggcgcccttctcccctgtctctgtgctgtagccgtcctggagttccatgatgaagccgtgggcattggccttctgtgcggcctccaccaccatctcgaaaggcacagtgggcaggccgtaggagatgttatccgtgatggagcgggcgaacagcacgggctcctggctcaccagggagatcacacggtgcaagtacttgtggtcgtaggcgctgatgggcttgccgtccagcagcacccggcccccctccagggggtagaagttctccaggatgttgacacaggagctcttcccactgcccgagggccccaccagggccgtcaccttgccgggggacaggctgaaggagacattctccatacaatctcccaggacaaactcgtagatgatgaaggcgatgaggttgccgctggtcatctggcctgagatgacaaggtggcccccgtagtagaggatgctgacctggaccaccagcagtgtgagcccgctgccccagacgtagtacatgtaggcagctgcctccttcctgttcagcttgtacacctgctgcagcttccgcaggtacacctctgcctcctcctcctcattggcgaagctccggacagtcttcatggcactgatggtctcctccgccgtgttgctcgctctggccagggcattctggacctctttggagagcctcttgtagtacttgccgtagatgttggacaccatcatgatgatggggaagcccatgaaggtgaccaaggagagctgccatgagaggctgaacatgaagaccaccacgcccgtgaccttgactgtgttccgcaggaagacattgatgttctgggagaccaggtcgctgaccatggtggtgtccgaggtcaggcgggagatgaggtcccctgtgcggttctcatcaaagaagcttgtctcctgggacaccagtgagcggaagagacagtttcgaaggcgaatgttcagtctggcaaatatgagggtaaaaatgccgccccgaatacctgcggcaaatgagctgccaatggccagcaggcacacgatgacgacagccgtgctgaactgatccatgcttttctggatgacgatgccatcaatggcgcggcccgtgtagtagggcaggaaggtctctcccagagctgccacgatgaggaagaaggaggcggccacgaggaaggccacgtcgggcttggtgtaggagagcagcttctgcagcgtggccccagacgcctgctcgggcggtggccggccgctcccagggaagccctcagcctcggtggccgcccctggctccagggcctgggtgcctggccgcacggtggacagcagccaccagagcaggaaggatgcgccgagtgaaatgtacgtccacacgaacagggcccaaaaccaggggtcccggatgggcctgcgcacctctgagaagagcagcagcttcaccatggcatagatgcccacgaagaggcacacgagggtgatgaccagccacgaggcccgcagccgccggggccccagcgcactgttcttggccacaccaatggtggctcccagcagcaggcagctgcggtacaggcaggctgcccagagatccagcaccgagtcaaagatgttgaagtggcggatgtcctccaggaggctgcggtccaggtggctgaagacatagatggccgtggtcacgcagatgtccacactcatgaaggccaaagtcaccaccaccgccttccacagccgcatcctgctggttggaggtgggcgggtgctgaaggccaggttgtagctcacgggggcaaggccatcatcatccacagggcgaggccaggcctgttacctggcaccaggtgagctctgggagggggcgcgcagcaggctcgggtctggggtgcagtttccgcgctgctcattgaagactgcgccggacgcggtcctcgctccgctcttcccgctgctcctccccgcctcccacccgcgctgcgccgctgcaaggtcggagctgagact

SEQ ID NO: 16082 - RNA, 3991 nt, Homo sapiens
  source 1..3991: mol_type = other RNA
gctgggattacaggcatgagccattgcacctggccacttacccattttaaagtgtacaaatgcattggtattaaatgtattcacaatattgtgcaaacaccaggtctctccagcttccaaactttctcatcaccctgtaaaaaacatcttgtatccagcaagcagtcactccccattcctccctccccatgccctggtaacctctaatctgctttctatccctatagatttgcttcttctgaatatatcatgtaaaaagaatcataccataggtgaccttccctgcctggcatctttcatttgcataatgcttctaaggaccatctatgttatagcatgtaccagcacttcattcctttctacagctgaatcatatcccacagtatgtgcataccacggtttgcagtttgtttatccattcatacattggattgtttgcactttttggctttattttattatttttagagacgaggtctcactctgtcatccaggctggagtgcagtggcaccaccatggttcgttgcagcctcaacctccttgagctcaaaggatcctcctgcctcagccacacaagtagctgggacgaccggtatgcactaccacgcctggctgatttttaaatttttgtagggatggggtcccactatgttgcccaggctgttctcaaactcctggcttcaagcaatcctcccgcctcagcctcccaaagtgctgggattacaactgtgagccactgtgcccaggtccatgttgagctttttgaggaagtgccagactgtggttgggatcattctttcctctagatacccaaagctggtacctccttgtcattcagggctcagctcccatatcacctccccagaccaccccagctcaaacagtgctcctctcccaagtcactctcttgtctgctgccatcttttcaccatctggagtttattacccagtaggatgtaggtgatctcggacctcttagtctccactgtgacccacaacctagcacagtttctggtagacggaggttctcaataaatgcttactgaatgactgatctcaggtagtcaaaggtaaagagctgtaataatgtgaggcactgtcactgtcaccttaggtcgctgttaggacctccccctgggtgactcatctgtttgtttgtttatttatttatttatttatttatttatttatttatttattttagatggagtctcactctgtcgtccaggctggagttcagaggcacaatctcggctcactgccacctctgcctcccgggttcaagtgattctcctgcctcagcctccccaccacacctggctaatttttgtgtttttagtagagatgagttttcaccatgttggccaggctggtctccaactcctgacctcaagtggtccgcctgcctcggcctcccaaagtgctgggattacaggcatgagccaccacgcccagccaactcacctgtttaaatggtcaacttcctcctctctgaggaaagaataaaaaccaggaaagagaaaccattggcgatgcttctttctcagccctttcctgttagtgactcagcacaggtatctccttcactatccccagctcctgaggtgcaacaagcagcccttagtgacaactgaatggttatcattgtcatcatcatcaatccatctcggttctgatatctgcaggctggtcattcagatcagatactcgctctcggcatccaaagcgctggtggcttcatccaggatgaggactggggggttccgcaccagagcccgggccatggccacccgctgcttctggccacctgacagctgggcgcccttctcccctgtctctgtgctgtagccgtcctggagttccatgatgaagccgtgggcattggccttctgtgcggcctccaccaccatctcgaaaggcacagtgggcaggccgtaggagatgttatccgtgatggagcgggcgaacagcacgggctcctggctcaccagggagatcacacggtgcaagtacttgtggtcgtaggcgctgatgggcttgccgtccagcagcacccggcccccctccagggggtagaagttctccaggatgttgacacaggagctcttcccactgcccgagggccccaccagggccgtcaccttgccgggggacaggctgaaggagacattctgcaggacctgggtgtggggccgagtgcggtaggtgaaggtcacattctcaaagtccacccggccctccaggtggtcgggggccaagctgccatcgtgcaccatggtcggctgccggtcgatgaactcgaacaccttctcagcagcccccactccctgcatcaggccactgtagacggagcccacggactccatacaatctcccaggacaaactcgtagatgatgaaggcgatgaggttgccgctggtcatctggcctgagatgacaaggtggcccccgtagtagaggatgctgacctggaccaccagcagtgtgagcccgctgccccagacgtagtacatgtaggcagctgcctccttcctgttcagcttgtacacctgctgcagcttccgcaggtacacctctgcctcctcctcctcattggcgaagctccggacagtcttcatggcactgatggtctcctccgccgtgttgctcgctctggccagggcattctggacctctttggagagcctcttgtagtacttgccgtagatgttggacaccatcatgatgatggggaagcccatgaaggtgaccaaggagagctgccatgagaggctgaacatgaagaccaccacgcccgtgaccttgactgtgttccgcaggaagacattgatgttctgggagaccaggtcgctgaccatggtggtgtccgaggtcaggcgggagatgaggtcccctgtgcggttctcatcaaagaagcttgtctcctgggacaccagtgagcggaagagacagtttcgaaggcgaatgttcagtctggcaaatatgagggtaaaaatgccgccccgaatacctgccaatggccagcaggcacacgatgacgacagccgtgctgaactgatccatgcttttctggatgacgatgccatcaatggcgcggcccgtgtagtagggcaggaaggtctctcccagagctgccacgatgaggaagaaggaggcggccacgaggaaggccacgtcgggcttggtgtaggagagcagcttctgcagcgtggccccagacgcctgctcgggcggtggccggccgctcccagggaagccctcagcctcggtggccgcccctggctccagggcctgggtgcctggccgcacggtggacagcagccaccagagcaggaaggatgcgccgagtgaaatgtacgtccacacgaacagggcccaaaaccaggggtcccggatgggcctgcgcacctctgagaagagcagcagcttcaccatggcatagatgcccacgaagaggcacacgagggtgatgaccagccacgaggcccgcagccgccggggccccagcgcactgttcttggccacaccaatggtggctcccagcagcaggcagctgcggtacaggcaggctgcccagagatccagcaccgagtcaaagatgttgaagtggcggatgtcctccaggaggctgcggtccaggtggctgaagacatagatggccgtggtcacgcagatgtccacactcatgaaggccaaagtcaccaccaccgccttccacagccgcatcctgctggttggaggtgggcgggtgctgaaggccaggttgtagctcacgggggcaaggccatcatcatccacagggcgaggccaggcctgttacctggcaccaggtgagctctgggagggggcgcgcagcaggctcgggtctggggtgcagtttccgcgctgctcattgaagactgcgccggacgcggtcctcgctccgctcttcccgctgctcctccccgcctcccacccgcgctgcgccgctgcaaggtcggagctgagact

SEQ ID NO: 16083 - RNA, 4005 nt, Homo sapiens
  source 1..4005: mol_type = other RNA
gctgggattacaggcatgagccattgcacctggccacttacccattttaaagtgtacaaatgcattggtattaaatgtattcacaatattgtgcaaacaccaggtctctccagcttccaaactttctcatcaccctgtaaaaaacatcttgtatccagcaagcagtcactccccattcctccctccccatgccctggtaacctctaatctgctttctatccctatagatttgcttcttctgaatatatcatgtaaaaagaatcataccataggtgaccttccctgcctggcatctttcatttgcataatgcttctaaggaccatctatgttatagcatgtaccagcacttcattcctttctacagctgaatcatatcccacagtatgtgcataccacggtttgcagtttgtttatccattcatacattggattgtttgcactttttggctttattttattatttttagagacgaggtctcactctgtcatccaggctggagtgcagtggcaccaccatggttcgttgcagcctcaacctccttgagctcaaaggatcctcctgcctcagccacacaagtagctgggacgaccggtatgcactaccacgcctggctgatttttaaatttttgtagggatggggtcccactatgttgcccaggctgttctcaaactcctggcttcaagcaatcctcccgcctcagcctcccaaagtgctgggattacaactgtgagccactgtgcccaggtccatgttgagctttttgaggaagtgccagactgtggttgggatcattctttcctctagatacccaaagctggtacctccttgtcattcagggctcagctcccatatcacctccccagaccaccccagctcaaacagtgctcctctcccaagtcactctcttgtctgctgccatcttttcaccatctggagtttattacccagtaggatgtaggtgatctcggacctcttagtctccactgtgacccacaacctagcacagtttctggtagacggaggttctcaataaatgcttactgaatgactgatctcaggtagtcaaaggtaaagagctgtaataatgtgaggcactgtcactgtcaccttaggtcgctgttaggacctccccctgggtgactcatctgtttgtttgtttatttatttatttatttatttatttatttatttatttattttagatggagtctcactctgtcgtccaggctggagttcagaggcacaatctcggctcactgccacctctgcctcccgggttcaagtgattctcctgcctcagcctccccaccacacctggctaatttttgtgtttttagtagagatgagttttcaccatgttggccaggctggtctccaactcctgacctcaagtggtccgcctgcctcggcctcccaaagtgctgggattacaggcatgagccaccacgcccagccaactcacctgtttaaatggtcaacttcctcctctctgaggaaagaataaaaaccaggaaagagaaaccattggcgatgcttctttctcagccctttcctgttagtgactcagcacaggtatctccttcactatccccagctcctgaggtgcaacaagcagcccttagtgacaactgaatggttatcattgtcatcatcatcaatccatctcggttctgatatctgcaggctggtcattcagatcagatactcgctctcggcatccaaagcgctggtggcttcatccaggatgaggactggggggttccgcaccagagcccgggccatggccacccgctgcttctggccacctgacagctgggcgcccttctcccctgtctctgtgctgtagccgtcctggagttccatgatgaagccgtgggcattggccttctgtgcggcctccaccaccatctcgaaaggcacagtgggcaggccgtaggagatgttatccgtgatggagcgggcgaacagcacgggctcctggctcaccagggagatcacacggtgcaagtacttgtggtcgtaggcgctgatgggcttgccgtccagcagcacccggcccccctccagggggtagaagttctccaggatgttgacacaggagctcttcccactgcccgagggccccaccagggccgtcaccttgccgggggacaggctgaaggagacattctgcaggacctgggtgtggggccgagtgcggtaggtgaaggtcacattctcaaagtccacccggccctccaggtggtcgggggccaagctgccatcgtgcaccatggtcggctgccggtcgatgaactcgaacaccttctcagcagcccccactccctgcatcaggccactgtagacggagcccacggactccatacaatctcccaggacaaactcgtagatgatgaaggcgatgaggttgccgctggtcatctggcctgagatgacaaggtggcccccgtagtagaggatgctgacctggaccaccagcagtgtgagcccgctgccccagacgtagtacatgtaggcagctgcctccttcctgttcagcttgtacacctgctgcagcttccgcaggtacacctctgcctcctcctcctcattggcgaagctccggacagtcttcatggcactgatggtctcctccgccgtgttgctcgctctggccagggcattctggacctctttggagagcctcttgtagtacttgccgtagatgttggacaccatcatgatgatggggaagcccatgaaggtgaccaaggagagctgccatgagaggctgaacatgaagaccaccacgcccgtgaccttgactgtgttccgcaggaagacattgatgttctgggagaccaggtcgctgaccatggtggtgtccgaggtcaggcgggagatgaggtcccctgtgcggttctcatcaaagaagcttgtctcctgggacaccagtgagcggaagagacagtttcgaaggcgaatgttcagtctggcaaatatgagggtaaaaatgccgccccgaatacctgcggcaaatgagctgccaatggccagcaggcacacgatgacgacagccgtgctgaactgatccatgcttttctggatgacgatgccatcaatggcgcggcccgtgtagtagggcaggaaggtctctcccagagctgccacgatgaggaagaaggaggcggccacgaggaaggccacgtcgggcttggtgtaggagagcagcttctgcagcgtggccccagacgcctgctcgggcggtggccggccgctcccagggaagccctcagcctcggtggccgcccctggctccagggcctgggtgcctggccgcacggtggacagcagccaccagagcaggaaggatgcgccgagtgaaatgtacgtccacacgaacagggcccaaaaccaggggtcccggatgggcctgcgcacctctgagaagagcagcagcttcaccatggcatagatgcccacgaagaggcacacgagggtgatgaccagccacgaggcccgcagccgccggggccccagcgcactgttcttggccacaccaatggtggctcccagcagcaggcagctgcggtacaggcaggctgcccagagatccagcaccgagtcaaagatgttgaagtggcggatgtcctccaggaggctgcggtccaggtggctgaagacatagatggccgtggtcacgcagatgtccacactcatgaaggccaaagtcaccaccaccgccttccacagccgcatcctgctggttggaggtgggcgggtgctgaaggccaggttgtagctcacgggggcaaggccatcatcatccacagggcgaggccaggcctgttacctggcaccaggtgagctctgggagggggcgcgcagcaggctcgggtctggggtgcagtttccgcgctgctcattgaagactgcgccggacgcggtcctcgctccgctcttcccgctgctcctccccgcctcccacccgcgctgcgccgctgcaaggtcggagctgagact

SEQ ID NO: 16084 - RNA, 2485 nt, Homo sapiens
  source 1..2485: mol_type = other RNA
gctgggattacaggcatgagccattgcacctggccacttacccattttaaagtgtacaaatgcattggtattaaatgtattcacaatattgtgcaaacaccaggtctctccagcttccaaactttctcatcaccctgtttaaatggtcaacttcctcctctctgaggaaagaataaaaaccaggaaagagaaaccattggcgatgcttctttctcagccctttcctgttagtgactcagcacaggtatctccttcactatccccagctcctgaggtgcaacaagcagcccttagtgacaactgaatggttatcattgtcatcatcatcaatccatctcggttctgatatctgcaggctggtcattcagatcagatactcgctctcggcatccaaagcgctggtggcttcatccaggatgaggactggggggttccgcaccagagcccgggccatggccacccgctgcttctggccacctgacagctgggcgcccttctcccctgtctctgtgctgtagccgtcctggagttccatgatgaagccgtgggcattggccttctgtgcggcctccaccaccatctcgaaaggcacagtgggcaggccgtaggagatgttatccgtgatggagcgggcgaacagcacgggctcctggctcaccagggagatcacacggtgcaagtacttgtggtcgtaggcgctgatgggcttgccgtccagcagcacccggcccccctccagggggtagaagttctccaggatgttgacacaggagctcttcccactgcccgagggccccaccagggccgtcaccttgccgggggacaggctgaaggagacattctccatacaatctcccaggacaaactcgtagatgatgaaggcgatgaggttgccgctggtcatctggcctgagatgacaaggtggcccccgtagtagaggatgctgacctggaccaccagcagtgtgagcccgctgccccagacgtagtacatgtaggcagctgcctccttcctgttcagcttgtacacctgctgcagcttccgcaggtacacctctgcctcctcctcctcattggcgaagctccggacagtcttcatggcactgatggtctcctccgccgtgttgctcgctctggccagggcattctggacctctttggagagcctcttgtagtacttgccgtagatgttggacaccatcatgatgatggggaagcccatgaaggtgaccaaggagagctgccatgagaggctgaacatgaagaccaccacgcccgtgaccttgactgtgttccgcaggaagacattgatgttctgggagaccaggtcgctgaccatggtggtgtccgaggtcaggcgggagatgaggtcccctgtgcggttctcatcaaagaagcttgtctcctgggacaccagtgagcggaagagacagtttcgaaggcgaatgttcagtctggcaaatatgagggtaaaaatgccgccccgaatacctgcggcaaatgagctgccaatggccagcaggcacacgatgacgacagccgtgctgaactgatccatgcttttctggatgacgatgccatcaatggcgcggcccgtgtagtagggcaggaaggtctctcccagagctgccacgatgaggaagaaggaggcggccacgaggaaggccacgtcgggcttggtgtaggagagcagcttctgcagcgtggccccagacgcctgctcgggcggtggccggccgctcccagggaagccctcagcctcggtggccgcccctggctccagggcctgggtgcctggccgcacggtggacagcagccaccagagcaggaaggatgcgccgagtgaaatgtacgtccacacgaacagggcccaaaaccaggggtcccggatgggcctgcgcacctctgagaagagcagcagcttcaccatggcatagatgcccacgaagaggcacacgagggtgatgaccagccacgaggcccgcagccgccggggccccagcgcactgttcttggccacaccaatggtggctcccagcagcaggcagctgcggtacaggcaggctgcccagagatccagcaccgagtcaaagatgttgaagtggcggatgtcctccaggaggctgcggtccaggtggctgaagacatagatggccgtggtcacgcagatgtccacactcatgaaggccaaagtcaccaccaccgccttccacagccgcatcctgctggttggaggtgggcgggtgctgaaggccaggttgtagctcacgggggcaaggccatcatcatccacagggcgaggccaggcctgttacctggcaccaggtgagctctgggagggggcgcgcagcaggctcgggtctggggtgcagtttccgcgctgctcattgaagactgcgccggacgcggtcctcgctccgctcttcccgctgctcctccccgcctcccacccgcgctgcgccgctgcaaggtcggagctgagact

SEQ ID NO: 16085 - RNA, 2674 nt, Homo sapiens
  source 1..2674: mol_type = other RNA
gctgggattacaggcatgagccattgcacctggccacttacccattttaaagtgtacaaatgcattggtattaaatgtattcacaatattgtgcaaacaccaggtctctccagcttccaaactttctcatcaccctgtttaaatggtcaacttcctcctctctgaggaaagaataaaaaccaggaaagagaaaccattggcgatgcttctttctcagccctttcctgttagtgactcagcacaggtatctccttcactatccccagctcctgaggtgcaacaagcagcccttagtgacaactgaatggttatcattgtcatcatcatcaatccatctcggttctgatatctgcaggctggtcattcagatcagatactcgctctcggcatccaaagcgctggtggcttcatccaggatgaggactggggggttccgcaccagagcccgggccatggccacccgctgcttctggccacctgacagctgggcgcccttctcccctgtctctgtgctgtagccgtcctggagttccatgatgaagccgtgggcattggccttctgtgcggcctccaccaccatctcgaaaggcacagtgggcaggccgtaggagatgttatccgtgatggagcgggcgaacagcacgggctcctggctcaccagggagatcacacggtgcaagtacttgtggtcgtaggcgctgatgggcttgccgtccagcagcacccggcccccctccagggggtagaagttctccaggatgttgacacaggagctcttcccactgcccgagggccccaccagggccgtcaccttgccgggggacaggctgaaggagacattctgcaggacctgggtgtggggccgagtgcggtaggtgaaggtcacattctcaaagtccacccggccctccaggtggtcgggggccaagctgccatcgtgcaccatggtcggctgccggtcgatgaactcgaacaccttctcagcagcccccactccctgcatcaggccactgtagacggagcccacggactccatacaatctcccaggacaaactcgtagatgatgaaggcgatgaggttgccgctggtcatctggcctgagatgacaaggtggcccccgtagtagaggatgctgacctggaccaccagcagtgtgagcccgctgccccagacgtagtacatgtaggcagctgcctccttcctgttcagcttgtacacctgctgcagcttccgcaggtacacctctgcctcctcctcctcattggcgaagctccggacagtcttcatggcactgatggtctcctccgccgtgttgctcgctctggccagggcattctggacctctttggagagcctcttgtagtacttgccgtagatgttggacaccatcatgatgatggggaagcccatgaaggtgaccaaggagagctgccatgagaggctgaacatgaagaccaccacgcccgtgaccttgactgtgttccgcaggaagacattgatgttctgggagaccaggtcgctgaccatggtggtgtccgaggtcaggcgggagatgaggtcccctgtgcggttctcatcaaagaagcttgtctcctgggacaccagtgagcggaagagacagtttcgaaggcgaatgttcagtctggcaaatatgagggtaaaaatgccgccccgaatacctgcggcaaatgagctgccaatggccagcaggcacacgatgacgacagccgtgctgaactgatccatgcttttctggatgacgatgccatcaatggcgcggcccgtgtagtagggcaggaaggtctctcccagagctgccacgatgaggaagaaggaggcggccacgaggaaggccacgtcgggcttggtgtaggagagcagcttctgcagcgtggccccagacgcctgctcgggcggtggccggccgctcccagggaagccctcagcctcggtggccgcccctggctccagggcctgggtgcctggccgcacggtggacagcagccaccagagcaggaaggatgcgccgagtgaaatgtacgtccacacgaacagggcccaaaaccaggggtcccggatgggcctgcgcacctctgagaagagcagcagcttcaccatggcatagatgcccacgaagaggcacacgagggtgatgaccagccacgaggcccgcagccgccggggccccagcgcactgttcttggccacaccaatggtggctcccagcagcaggcagctgcggtacaggcaggctgcccagagatccagcaccgagtcaaagatgttgaagtggcggatgtcctccaggaggctgcggtccaggtggctgaagacatagatggccgtggtcacgcagatgtccacactcatgaaggccaaagtcaccaccaccgccttccacagccgcatcctgctggttggaggtgggcgggtgctgaaggccaggttgtagctcacgggggcaaggccatcatcatccacagggcgaggccaggcctgttacctggcaccaggtgagctctgggagggggcgcgcagcaggctcgggtctggggtgcagtttccgcgctgctcattgaagactgcgccggacgcggtcctcgctccgctcttcccgctgctcctccccgcctcccacccgcgctgcgccgctgcaaggtcggagctgagact

SEQ ID NO: 16086 - RNA, 1970 nt, Homo sapiens
  source 1..1970: mol_type = other RNA
gctgggattacaggcatgagccattgcactcagcccagatatcactttaaaaagggaaaataacagacacaatgtctggcataaacctagactggaaaaaggcaaagctgtatggtcaacatgaaacataggagaaggtactaacagtcccagggaagcagggagggaggccacaggggagaagtccagggacatgagttcgctgtttcccaagggaaaccagtgccttcaggccactctgtatgggagatcctgtagcagactctggaactgcaaccaaagcatgagtgggaagtcaggcaaattcaggttgataattgattggtttccttgggcaagtaccttacatctcccagccaggtgctcagccatgaaagcgggttaatcgtagccatttcacaggttgttgtaaaagttaaattagaaaacctgcctaaacaaatgcctggccagggtcgatgttcaaaggtaagaagagtgaggggccggcagggcatccagtccggccccaagcagcttggaggtggcaggaaaactgtgtttgtacatttccccttatgaacttctatcccaggatggagacaacctctttgaagagcagtgcctagaatggcctcccaggaccacatctccatcacagctggaatctcatccgtcatctctgcagcagggtcagaaactggctgcggcaagcaaggttcatttcaccctcttcctcagcaagagaagccccagctgcttcttttctggcatttccctgtgcctactggttgggatggccagcagcagagtatttggcctccgaccacctagaaaaagccatgccttggttaagaagtgctgcatttgagaatatggacctttgtggttccccgtatccctgggaacctccacattcagagaggctaaaagcccacaccgacccgagccaacagaatggggaggaagcaggtgcagggagtcagcttcatcttccccttctcttgatgatgctcttcagccattagggtttcaaaagagtgggcgtgagcaagcgagaaaagccccttcaattctgggaaacttaaagacagtttcttccagcaggaacacctgggtctgttagacggtgcggtgcctgcagctgatttgatgggttggaaatgcgcacgaaacaaaatacttgaatcctggaaatggttattttgtgtcttttcccttgaatatattattaaatccccaagaacaggaattggctcttactcatcttcatgtttctccagccaccagcccaggttttactcatagtaggtgctcacaataaatgcacaaagatagatgtataaggactttccatgcagcatttccatgcagtgtcggcaccacgctggaaatgtcgtaaacacttatcagtagggatttatgtccaggcatcagcttcatgggtgtgtagcagcagcttcctcatccctgggttgcagccacgaactcaacaaccccaatggcggctcctgcttccccctctcactgaccatggcagagggagcagctccctgagaggcctgtatggtggaagagttctgggagtcccttctggaaacccaacctggagctcactcctctggtccatccagtgatttggtaaatttctgagttctagaacataccaccatggctgtgatcctaggaacaggatgcccccagcacccagaatactggcagctagacataggaaagtcttctgctgcagcagcatgagctgcctgcaggaagtagccaggagcatttgcagggacttctgcctctgactgtcttccaggtcatgtgcaaacacttgtggaaggtccagcaagaacaaggtaacctgtgttctcccgggtgtaaaccgcgtctctgtgaagggaaagggggaagagggccggcaaggacctccagtatcagcgaggactatcaggacgtccagctaataaacgactttttcactgtccaca

SEQ ID NO: 16087 - RNA, 1037 nt, Homo sapiens
  source 1..1037: mol_type = other RNA
gctgggattacaggcatgagccattgcccaaagtataaccttatgtcagtaattgctataaaatataatcagcattgtaatagcaatctaacaaattctggtcaacagggcagtctgctatttgaaattacccttgggttgcatcttacaaaaggcttatattaaaatcagcaaagatgaaaattgtgtgtagtcaaaattaccctttaaaaaaatctctatattaaagtatggttttgtgtacactatactgcgttacaatacgtccacccagtttctcctccaggttttaagcagcttactgtttctttggtttagcaccacacgaactaggcatcttacatttttaagctgtatagtacaaaaaagtatttgtaaacacataaatttgcgtaagctaagtgtgcatatgtgcacgtgtagtatatcacattgtaataacaaagcatggctttctaataaacctgtttgaattgggagaaataatgaaaaaacatttatgaaaacaatgacaaatatggttgcagtagatacactaaagcaaatatggacagtaaagaacattaaagttaacgatgatttttattagtacccaaaagcaaattcatatacactagatgattatcttacaaaactataacatgcccagaatgtcagttatttatcatgaaacaggtgattcctatgacaatggtggaaatgattaagaatcacactattaaaaacttatgactgcacagttaagccataaaagaaactttaagtttttagtgcattttcacattgatttttaaatcctgacaatgatcctagaaggaagatatctatttttatgtgtaaatatcaaagccaaggacatagagtttaaatgacttaccgaagatcacgcagcttgttagtgacagagcagggattagaaaccgggtctcttgattccccgtccagtgccacacaatgacggctttcaaagcgcctccacctctgcctccgcctccgcccctgccccggcaaccagctcaggacaagcgatgctcctc

SEQ ID NO: 16088 - RNA, 3559 nt, Homo sapiens
  source 1..3559: mol_type = other RNA
gctgggattacaggcatgagccattgcgcccggcctgccccatgtaactgagaaattctacttggtcatttcaatggaatgtgttattaaaacatacggtcaatatgcatattgtaaaattatagtatagtcaaaataattaggtacatatcagaaacataatccactttatctgatctggttaggaccagcgcttgtgaacttcaacatataccttgccaaatggttgaaatatttgtgttttaaacactattacataggaaacccactgatacttatattttctacaaccatttatagctgggtttatatatggtaacttttctgaattccatattgagacacgggttggacaagtgtgactatacttaccgggcaatacaacaggatatctgaaagcaggttagttcagtttgataattgcttagcccagttttgaaaaacctgccttccttttgaatattttgattaattttgcagaatagatccttttgactctaagagagaagggaacgcaataccagcaaaagattttttcctattttgtgtcatgtaacatgaatggtatgtggtcaagcaggtgtgtaacttaccgggtactatagtatccagtgaaatacaagtcaattcttaaattctcctgcaatttataatgctaacatttacaaatgacatactcaaaatttcataggaggacactaatctgtggcacagtccaatcaggctaatgcatttggaaaatgcattttttatatatatgtagatagattacatatacatgtctatacgtgtgtatatatatttttctatatatatttaaaagactagtgtagtttaaaaatttacttataaatttacttataagatgaatcgtagggagttaggaaagattgctttcatatgctttaattctcagattgaagatactctgatatttaaataaacatactttgcattgtcagaaagataacttttcccagagaggatttgactttaatagtctagattagctgcctaagtcaacagtcactgaaataacattgttttcttatctttatctacacttgtggcctatcatcagtgacctttgtcacttctcttgctgtccctccctctgtatttcacctctatggatgactgccagttcctaatctttttcctagccccatcttccattaggactggtttttatccaaaatgtaccgacttgaaatggaaactttttttgatagctttctctttgacttttagtttcagctcctgctcactcaggcctgctatgtaacctgtacttatttacccttactgtgttttcccttctcggctaaaaggaaccaagttactttctctgtggtcactgagtggtgaggttattttgggccatgagggctgggggcagggttaggctggggaggtagctgaaataagtttcatggctgaagctcatctttggttttcaagtctcataggccttgcaatctaattctcattaggaatagaattaatttgtgtacctaacatgtcatctggttgtttactatttgaaacaactgaaacacatcagtgcttctggagggatagtatttcgttctactcttggttccacattttacaaattacattccctgcatttttaattaagtaaaagggctgagaaaggtcacttttcttcctttatatttaaaaaacaaaccaactctaagtctgttaagtttcagatacaaaaatcatcctgaaattaccatgacataactaaaaacaattctgccagaattaaggacagagaggaaaacctataactatcaggaagaacaaatgtttatctgaaacaacaggtaaccttgggaaggtatcaactatgaattttagaaccaaagaactttggatataaggaggaagtgtgtgcatggctaatagacaaggcagagaaaagcagttattaatccagagtagcaagtctacccaatcagtgagcaaactgagaggtccaccagacattaattttaatgaggttactcaagatttcccctttcttcaagcattccaggaatcagatggaggaagatagggtaacatcatctttatcaaatatttgcaaacattatatagatagctggaaaagcctgtgcatggtgaatggaagagatgtcacataaaaccgaataactgagtctcataatatttaggtcttgaatgaagttaggccttgatctgcttccagccagttgatctcttaattatgtaggctgtgcaacaagtttttggttctgttttatagttttcttctctgcattcctctagatttaatatattcttgatttgttttacagatcactgcttttcctccagaataagccaatgtggataagggagaccaaaggaaattaattatataccaataagaaaagtcttacgtaaaccctgtgtgtaataaatgttcaaataagttggttgtaaggttttggtgtacaatttcaagatattttcacagaacatattgctccccagtcagggttaaagtgaaacgttccatggggataatgcagaggatgatattctttcaggaaaaagagtattaagctttcctctactaggcatcttccctcaggcactgagattgcagccatccaacaaatggggaagggcagaaagaggagccttcaaaagtcgcaaatatacttcaatagctactttttagcaagtgtggtaatgagatctttccattctcccctcttctttgtgatgtatgcaggggtgagtagctgcagcagtgattctgtctgttgcctaaagaagttctgacacaaggcctcagtgttacatatcacgtacatcccacagtcatagctgttttgttgggcaggggctttctcttccacaaaggccagtttgtctccttttctgcctaagaaagcctccagtttctctgctacctgctttgcgtgaactgagttgctcctgctatgggaatcataatgaaaaaagctatttttatcttggaggtagaccaataaactccagtgggttcctccagctgcctggttggagttatcattgatggctaaaaatacaactctcttgttggggaggtccagtggttcaaggaacatggcaatctctgctgggttgctagtgcacttgatgaactgggtgacttcagggctgatgaaactgacgtgatcagagcagtcatgaaactgactgttggcaaagtactcaaacgcaaacccaataatatggtcattgagccagcttggcggatccaatagtgagacatctgattgccgcagtagactgtccatgtaactcaagactacggggtccatcttgtactgacgagggctgctcagaaattccagaagctgaacaagagacatggattttcttttgcctctgccacccctgagacagcaagaccaattgctccttttcctcctcctcttcagcctactcaacatgatgatgaggatgaagacctttatgacgatccatttccactgcctcgggcctcaccaccccaaccagccttcaggcacctctgtgttggccggaaagcgac

SEQ ID NO: 16089 - RNA, 3536 nt, Homo sapiens
  source 1..3536: mol_type = other RNA
gctgggattacaggcatgagccattgcgcccggcctgccccatgtaactgagaaattctacttggtcatttcaatggaatgtgttattaaaacatacggtcaatatgcatattgtaaaattatagtatagtcaaaataattaggtacatatcagaaacataatccactttatctgatctggttaggaccagcgcttgtgaacttcaacatataccttgccaaatggttgaaatatttgtgttttaaacactattacataggaaacccactgatacttatattttctacaaccatttatagctgggtttatatatggtaacttttctgaattccatattgagacacgggttggacaagtgtgactatacttaccgggcaatacaacaggatatctgaaagcaggttagttcagtttgataattgcttagcccagttttgaaaaacctgccttccttttgaatattttgattaattttgcagaatagatccttttgactctaagagagaagggaacgcaataccagcaaaagattttttcctattttgtgtcatgtaacatgaatggtatgtggtcaagcaggtgtgtaacttaccgggtactatagtatccagtgaaatacaagtcaattcttaaattctcctgcaatttataatgctaacatttacaaatgacatactcaaaatttcataggaggacactaatctgtggcacagtccaatcaggctaatgcatttggaaaatgcattttttatatatatgtagatagattacatatacatgtctatacgtgtgtatatatatttttctatatatatttaaaagactagtgtagtttaaaaatttacttataaatttacttataagatgaatcgtagggagttaggaaagattgctttcatatgctttaattctcagattgaagatactctgatatttaaataaacatactttgcattgtcagaaagataacttttcccagagaggatttgactttaatagtctagattagctgcctaagtcaacagtcactgaaataacattgttttcttatctttatctacacttgtggcctatcatcagtgacctttgtcacttctcttgctgtccctccctctgtatttcacctctatggatgactgccagttcctaatctttttcctagccccatcttccattaggactggtttttatccaaaatgtaccgacttgaaatggaaactttttttgatagctttctctttgacttttagtttcagctcctgctcactcaggcctgctatgtaacctgtacttatttacccttactgtgttttcccttctcggctaaaaggaaccaagttactttctctgtggtcactgagtggtgaggttattttgggccatgagggctgggggcagggttaggctggggaggtagctgaaataagtttcatggctgaagctcatctttggttttcaagtctcataggccttgcaatctaattctcattaggaatagaattaatttgtgtacctaacatgtcatctggttgtttactatttgaaacaactgaaacacatcagtgcttctggagggatagtatttcgttctactcttggttccacattttacaaattacattccctgcatttttaattaagtaaaagggctgagaaaggtcacttttcttcctttatatttaaaaaacaaaccaactctaagtctgttaagtttcagatacaaaaatcatcctgaaattaccatgacataactaaaaacaattctgccagaattaaggacagagaggaaaacctataactatcaggaagaacaaatgtttatctgaaacaacaggtaaccttgggaaggtatcaactatgaattttagaaccaaagaactttggatataaggaggaagtgtgtgcatggctaatagacaaggcagagaaaagcagttattaatccagagtagcaagtctacccaatcagtgagcaaactgagaggtccaccagacattaattttaatgaggttactcaagatttcccctttcttcaagcattccaggaatcagatggaggaagatagggtaacatcatctttatcaaatatttgcaaacattatatagatagctggaaaagcctgtgcatggtgaatggaagagatgtcacataaaaccgaataactgagtctcataatatttaggtcttgaatgaagttaggccttgatctgcttccagccagttgatctcttaattatgtaggctgtgcaacaagtttttggttctgttttatagttttcttctctgcattcctctagatttaatatattcttgatttgttttacagatcactgcttttcctccagaataagccaatgtggataagggagaccaaaggaaattaattatataccaataagaaaagtcttacgtaaaccctgtgtgtaataaatgttcaaataagttggttgtaaggttttggtgtacaatttcaagatattttcacagaacatattgctccccagtcagggttaaagtgaaacgttccatggggataatgcagaggatgatattctttcaggaaaaagagtattaagctttcctctactaggcatcttccctcaggcactgagattgcagccatccaacaaatggggaagggcagaaagaggagccttcaaaagtcgcaaatatacttcaatagctactttttagcaagtgtggtaatgagatctttccattctcccctcttctttgtgatgtatgcaggggtgagtagctgcagcagtgattctgtctgttgcctaaagaagttctgacacaaggcctcagtgttacatatcacgtacatcccacagtcatagctgttttgttgggcaggggctttctcttccacaaaggccagtttgtctccttttctgcctaagaaagcctccagtttctctgctacctgctttgcgtgaactgagttgctcctgctatgggaatcataatgaaaaaagctatttttatcttggaggtagaccaataaactccagtgggttcctccagctgcctggttggagttatcattgatggctaaaaatacaactctcttgttggggaggtccagtggttcaaggaacatggcaatctctgctgggttgctagtgcacttgatgaactgggtgacttcagggctgatgaaactgacgtgatcagagcagtcatgaaactgactgttggcaaagtactcaaacgcaaacccaataatatggtcattgagccagcttggcggatccaatagtgagacatctgattgccgcagtagactgtccatgtaactcaagactacggggtccatcttgtactgacgagggctgctcagaaattccagaagctgaacaagagcctagccatcacggctttcagatagccgctgtcatggtgttcttactcccggtagatgtggtgtcagtccctctagacaccgtcacagactttggcttctctcccaccaccgactgtagcctctctcaacagacctctcctcaagcaaaccttgttatctttc

SEQ ID NO: 16090 - RNA, 3435 nt, Homo sapiens
  source 1..3435: mol_type = other RNA
gctgggattacaggcatgagccattgcgcccggcctgccccatgtaactgagaaattctacttggtcatttcaatggaatgtgttattaaaacatacggtcaatatgcatattgtaaaattatagtatagtcaaaataattaggtacatatcagaaacataatccactttatctgatctggttaggaccagcgcttgtgaacttcaacatataccttgccaaatggttgaaatatttgtgttttaaacactattacataggaaacccactgatacttatattttctacaaccatttatagctgggtttatatatggtaacttttctgaattccatattgagacacgggttggacaagtgtgactatacttaccgggcaatacaacaggatatctgaaagcaggttagttcagtttgataattgcttagcccagttttgaaaaacctgccttccttttgaatattttgattaattttgcagaatagatccttttgactctaagagagaagggaacgcaataccagcaaaagattttttcctattttgtgtcatgtaacatgaatggtatgtggtcaagcaggtgtgtaacttaccgggtactatagtatccagtgaaatacaagtcaattcttaaattctcctgcaatttataatgctaacatttacaaatgacatactcaaaatttcataggaggacactaatctgtggcacagtccaatcaggctaatgcatttggaaaatgcattttttatatatatgtagatagattacatatacatgtctatacgtgtgtatatatatttttctatatatatttaaaagactagtgtagtttaaaaatttacttataaatttacttataagatgaatcgtagggagttaggaaagattgctttcatatgctttaattctcagattgaagatactctgatatttaaataaacatactttgcattgtcagaaagataacttttcccagagaggatttgactttaatagtctagattagctgcctaagtcaacagtcactgaaataacattgttttcttatctttatctacacttgtggcctatcatcagtgacctttgtcacttctcttgctgtccctccctctgtatttcacctctatggatgactgccagttcctaatctttttcctagccccatcttccattaggactggtttttatccaaaatgtaccgacttgaaatggaaactttttttgatagctttctctttgacttttagtttcagctcctgctcactcaggcctgctatgtaacctgtacttatttacccttactgtgttttcccttctcggctaaaaggaaccaagttactttctctgtggtcactgagtggtgaggttattttgggccatgagggctgggggcagggttaggctggggaggtagctgaaataagtttcatggctgaagctcatctttggttttcaagtctcataggccttgcaatctaattctcattaggaatagaattaatttgtgtacctaacatgtcatctggttgtttactatttgaaacaactgaaacacatcagtgcttctggagggatagtatttcgttctactcttggttccacattttacaaattacattccctgcatttttaattaagtaaaagggctgagaaaggtcacttttcttcctttatatttaaaaaacaaaccaactctaagtctgttaagtttcagatacaaaaatcatcctgaaattaccatgacataactaaaaacaattctgccagaattaaggacagagaggaaaacctataactatcaggaagaacaaatgtttatctgaaacaacaggtaaccttgggaaggtatcaactatgaattttagaaccaaagaactttggatataaggaggaagtgtgtgcatggctaatagacaaggcagagaaaagcagttattaatccagagtagcaagtctacccaatcagtgagcaaactgagaggtccaccagacattaattttaatgaggttactcaagatttcccctttcttcaagcattccaggaatcagatggaggaagatagggtaacatcatctttatcaaatatttgcaaacattatatagatagctggaaaagcctgtgcatggtgaatggaagagatgtcacataaaaccgaataactgagtctcataatatttaggtcttgaatgaagttaggccttgatctgcttccagccagttgatctcttaattatgtaggctgtgcaacaagtttttggttctgttttatagttttcttctctgcattcctctagatttaatatattcttgatttgttttacagatcactgcttttcctccagaataagccaatgtggataagggagaccaaaggaaattaattatataccaataagaaaagtcttacgtaaaccctgtgtgtaataaatgttcaaataagttggttgtaaggttttggtgtacaatttcaagatattttcacagaacatattgctccccagtcagggttaaagtgaaacgttccatggggataatgcagaggatgatattctttcaggaaaaagagtattaagctttcctctactaggcatcttccctcaggcactgagattgcagccatccaacaaatggggaagggcagaaagaggagccttcaaaagtcgcaaatatacttcaatagctactttttagcaagtgtggtaatgagatctttccattctcccctcttctttgtgatgtatgcaggggtgagtagctgcagcagtgattctgtctgttgcctaaagaagttctgacacaaggcctcagtgttacatatcacgtacatcccacagtcatagctgttttgttgggcaggggctttctcttccacaaaggccagtttgtctccttttctgcctaagaaagcctccagtttctctgctacctgctttgcgtgaactgagttgctcctgctatgggaatcataatgaaaaaagctatttttatcttggaggtagaccaataaactccagtgggttcctccagctgcctggttggagttatcattgatggctaaaaatacaactctcttgttggggaggtccagtggttcaaggaacatggcaatctctgctgggttgctagtgcacttgatgaactgggtgacttcagggctgatgaaactgacgtgatcagagcagtcatgaaactgactgttggcaaagtactcaaacgcaaacccaataatatggtcattgagccagcttggcggatccaatagtgagacatctgattgccgcagtagactgtccatgtaactcaagactacggggtccatcttgtactgacgagggctgctcagaaattccagaagctgaacaagagctgcctcgggcctcaccaccccaaccagccttcaggcacctctgtgttggccggaaagcgac

SEQ ID NO: 16091 - RNA, 3659 nt, Homo sapiens
  source 1..3659: mol_type = other RNA
gctgggattacaggcatgagccattgcgcccggcctgccccatgtaactgagaaattctacttggtcatttcaatggaatgtgttattaaaacatacggtcaatatgcatattgtaaaattatagtatagtcaaaataattaggtacatatcagaaacataatccactttatctgatctggttaggaccagcgcttgtgaacttcaacatataccttgccaaatggttgaaatatttgtgttttaaacactattacataggaaacccactgatacttatattttctacaaccatttatagctgggtttatatatggtaacttttctgaattccatattgagacacgggttggacaagtgtgactatacttaccgggcaatacaacaggatatctgaaagcaggttagttcagtttgataattgcttagcccagttttgaaaaacctgccttccttttgaatattttgattaattttgcagaatagatccttttgactctaagagagaagggaacgcaataccagcaaaagattttttcctattttgtgtcatgtaacatgaatggtatgtggtcaagcaggtgtgtaacttaccgggtactatagtatccagtgaaatacaagtcaattcttaaattctcctgcaatttataatgctaacatttacaaatgacatactcaaaatttcataggaggacactaatctgtggcacagtccaatcaggctaatgcatttggaaaatgcattttttatatatatgtagatagattacatatacatgtctatacgtgtgtatatatatttttctatatatatttaaaagactagtgtagtttaaaaatttacttataaatttacttataagatgaatcgtagggagttaggaaagattgctttcatatgctttaattctcagattgaagatactctgatatttaaataaacatactttgcattgtcagaaagataacttttcccagagaggatttgactttaatagtctagattagctgcctaagtcaacagtcactgaaataacattgttttcttatctttatctacacttgtggcctatcatcagtgacctttgtcacttctcttgctgtccctccctctgtatttcacctctatggatgactgccagttcctaatctttttcctagccccatcttccattaggactggtttttatccaaaatgtaccgacttgaaatggaaactttttttgatagctttctctttgacttttagtttcagctcctgctcactcaggcctgctatgtaacctgtacttatttacccttactgtgttttcccttctcggctaaaaggaaccaagttactttctctgtggtcactgagtggtgaggttattttgggccatgagggctgggggcagggttaggctggggaggtagctgaaataagtttcatggctgaagctcatctttggttttcaagtctcataggccttgcaatctaattctcattaggaatagaattaatttgtgtacctaacatgtcatctggttgtttactatttgaaacaactgaaacacatcagtgcttctggagggatagtatttcgttctactcttggttccacattttacaaattacattccctgcatttttaattaagtaaaagggctgagaaaggtcacttttcttcctttatatttaaaaaacaaaccaactctaagtctgttaagtttcagatacaaaaatcatcctgaaattaccatgacataactaaaaacaattctgccagaattaaggacagagaggaaaacctataactatcaggaagaacaaatgtttatctgaaacaacaggtaaccttgggaaggtatcaactatgaattttagaaccaaagaactttggatataaggaggaagtgtgtgcatggctaatagacaaggcagagaaaagcagttattaatccagagtagcaagtctacccaatcagtgagcaaactgagaggtccaccagacattaattttaatgaggttactcaagatttcccctttcttcaagcattccaggaatcagatggaggaagatagggtaacatcatctttatcaaatatttgcaaacattatatagatagctggaaaagcctgtgcatggtgaatggaagagatgtcacataaaaccgaataactgagtctcataatatttaggtcttgaatgaagttaggccttgatctgcttccagccagttgatctcttaattatgtaggctgtgcaacaagtttttggttctgttttatagttttcttctctgcattcctctagatttaatatattcttgatttgttttacagatcactgcttttcctccagaataagccaatgtggataagggagaccaaaggaaattaattatataccaataagaaaagtcttacgtaaaccctgtgtgtaataaatgttcaaataagttggttgtaaggttttggtgtacaatttcaagatattttcacagaacatattgctccccagtcagggttaaagtgaaacgttccatggggataatgcagaggatgatattctttcaggaaaaagagtattaagctttcctctactaggcatcttccctcaggcactgagattgcagccatccaacaaatggggaagggcagaaagaggagccttcaaaagtcgcaaatatacttcaatagctactttttagcaagtgtggtaatgagatctttccattctcccctcttctttgtgatgtatgcaggggtgagtagctgcagcagtgattctgtctgttgcctaaagaagttctgacacaaggcctcagtgttacatatcacgtacatcccacagtcatagctgttttgttgggcaggggctttctcttccacaaaggccagtttgtctccttttctgcctaagaaagcctccagtttctctgctacctgctttgcgtgaactgagttgctcctgctatgggaatcataatgaaaaaagctatttttatcttggaggtagaccaataaactccagtgggttcctccagctgcctggttggagttatcattgatggctaaaaatacaactctcttgttggggaggtccagtggttcaaggaacatggcaatctctgctgggttgctagtgcacttgatgaactgggtgacttcagggctgatgaaactgacgtgatcagagcagtcatgaaactgactgttggcaaagtactcaaacgcaaacccaataatatggtcattgagccagcttggcggatccaatagtgagacatctgattgccgcagtagactgtccatgtaactcaagactacggggtccatcttgtactgacgagggctgctcagaaattccagaagctgaacaagagcttgattaatggcaccactctttcctcatgaaaccttcaggaacctgggaattgccctccgcttcactctgtacttcactgccaacatccagtctgtcactgccttgtacattttccctcatgatatttcaggtcattccttattactttttgttgcctctatcttattttaactgaaaatatctgtttgttgggcttctgtaatgctgagtggtcttcttgccttctgtcttctgcctcttgtcatgccctcctgttcattctcttgactgctgttggagtaagt

SEQ ID NO: 16092 - RNA, 3428 nt, Homo sapiens
  source 1..3428: mol_type = other RNA
gctgggattacaggcatgagccattgcgcccggcctgccccatgtaactgagaaattctacttggtcatttcaatggaatgtgttattaaaacatacggtcaatatgcatattgtaaaattatagtatagtcaaaataattaggtacatatcagaaacataatccactttatctgatctggttaggaccagcgcttgtgaacttcaacatataccttgccaaatggttgaaatatttgtgttttaaacactattacataggaaacccactgatacttatattttctacaaccatttatagctgggtttatatatggtaacttttctgaattccatattgagacacgggttggacaagtgtgactatacttaccgggcaatacaacaggatatctgaaagcaggttagttcagtttgataattgcttagcccagttttgaaaaacctgccttccttttgaatattttgattaattttgcagaatagatccttttgactctaagagagaagggaacgcaataccagcaaaagattttttcctattttgtgtcatgtaacatgaatggtatgtggtcaagcaggtgtgtaacttaccgggtactatagtatccagtgaaatacaagtcaattcttaaattctcctgcaatttataatgctaacatttacaaatgacatactcaaaatttcataggaggacactaatctgtggcacagtccaatcaggctaatgcatttggaaaatgcattttttatatatatgtagatagattacatatacatgtctatacgtgtgtatatatatttttctatatatatttaaaagactagtgtagtttaaaaatttacttataaatttacttataagatgaatcgtagggagttaggaaagattgctttcatatgctttaattctcagattgaagatactctgatatttaaataaacatactttgcattgtcagaaagataacttttcccagagaggatttgactttaatagtctagattagctgcctaagtcaacagtcactgaaataacattgttttcttatctttatctacacttgtggcctatcatcagtgacctttgtcacttctcttgctgtccctccctctgtatttcacctctatggatgactgccagttcctaatctttttcctagccccatcttccattaggactggtttttatccaaaatgtaccgacttgaaatggaaactttttttgatagctttctctttgacttttagtttcagctcctgctcactcaggcctgctatgtaacctgtacttatttacccttactgtgttttcccttctcggctaaaaggaaccaagttactttctctgtggtcactgagtggtgaggttattttgggccatgagggctgggggcagggttaggctggggaggtagctgaaataagtttcatggctgaagctcatctttggttttcaagtctcataggccttgcaatctaattctcattaggaatagaattaatttgtgtacctaacatgtcatctggttgtttactatttgaaacaactgaaacacatcagtgcttctggagggatagtatttcgttctactcttggttccacattttacaaattacattccctgcatttttaattaagtaaaagggctgagaaaggtcacttttcttcctttatatttaaaaaacaaaccaactctaagtctgttaagtttcagatacaaaaatcatcctgaaattaccatgacataactaaaaacaattctgccagaattaaggacagagaggaaaacctataactatcaggaagaacaaatgtttatctgaaacaacaggtaaccttgggaaggtatcaactatgaattttagaaccaaagaactttggatataaggaggaagtgtgtgcatggctaatagacaaggcagagaaaagcagttattaatccagagtagcaagtctacccaatcagtgagcaaactgagaggtccaccagacattaattttaatgaggttactcaagatttcccctttcttcaagcattccaggaatcagatggaggaagatagggtaacatcatctttatcaaatatttgcaaacattatatagatagctggaaaagcctgtgcatggtgaatggaagagatgtcacataaaaccgaataactgagtctcataatatttaggtcttgaatgaagttaggccttgatctgcttccagccagttgatctcttaattatgtaggctgtgcaacaagtttttggttctgttttatagttttcttctctgcattcctctagatttaatatattcttgatttgttttacagatcactgcttttcctccagaataagccaatgtggataagggagaccaaaggaaattaattatataccaataagaaaagtcttacgtaaaccctgtgtgtaataaatgttcaaataagttggttgtaaggttttggtgtacaatttcaagatattttcacagaacatattgctccccagtcagggttaaagtgaaacgttccatggggataatgcagaggatgatattctttcaggaaaaagagtattaagctttcctctactaggcatcttccctcaggcactgagattgcagccatccaacaaatggggaagggcagaaagaggagccttcaaaagtcgcaaatatacttcaatagctactttttagcaagtgtggtaatgagatctttccattctcccctcttctttgtgatgtatgcaggggtgagtagctgcagcagtgattctgtctgttgcctaaagaagttctgacacaaggcctcagtgttacatatcacgtacatcccacagtcatagctgttttgttgggcaggggctttctcttccacaaaggccagtttgtctccttttctgcctaagaaagcctccagtttctctgctacctgctttgcgtgaactgagttgctcctgctatgggaatcataatgaaaaaagctatttttatcttggaggtagaccaataaactccagtgggttcctccagctgcctggttggagttatcattgatggctaaaaatacaactctcttgttggggaggtccagtggttcaaggaacatggcaatctctgctgggttgctagtgcacttgatgaactgggtgacttcagggctgatgaaactgacgtgatcagagcagtcatgaaactgactgttggcaaagtactcaaacgcaaacccaataatatggtcattgagccagcttggcggatccaatagtgagacatctgattgccgcagtagactgtccatgtaactcaagactacggggtccatcttgtactgacgagggctgctcagaaattccagaagctgaacaagagcttgttatctttctccttagtcgcgatcctttctttggttgaaagggctttgcca

SEQ ID NO: 16093 - RNA, 2649 nt, Homo sapiens
  source 1..2649: mol_type = other RNA
gctgggattacaggcatgagccattgcgcctggcctctttctttactcctaatccatgatttgagagactcaaaccagccagaaagactctcagggatctggcgtcttaaggttcgggttcttctcttcacagtgaattcaaaaaagcctctgtctcctgacagaccccaaactttaaaaaaaaaaaaaaagcctctgtctttttgctttggcaaagcctggcagggggttagaaagccactgattccaggacaatacaagcttaagctcaagaggccagagatggggataggaagaaggcctaatgaggtggatagttctagaaatcagaaagaatgctgaataggtgaagtctgagtggtgacaacctcactgtcctgtctgcctcacaggagcagttctctacaaggctcttccacacacacacacgcaaggctcaggggctcggtgggtacaaaaagccagtggaaacggataaatacctatagcgttaatagcagaagtatgtccaaggttttgcacagggtaatcaaactaactggcttcagacatttgcagccacaggaaaaaatagctctcagccttatgagatggacattcctatactaactcccgctctttgttgtattgaattctggctgtttcttcccccactcaactgtgagcagatgtgcacagactccgagaggcagacaccaggaggtccagggacataggttggtgaggcatggcggtctagttgtgggagataatgaggcccagaaggtgtggtgagagacatggtggtgtgggaagttgagttgtgtttggggtggtattgggtgatggacaaggacagcagtcagcagagccttcgacccagcccaagcaggcaccccattgtgcttaggttcctatctgtggtcttgatttggctttgcttttcttgggaggaagatgaatcagaatcctggcatcgtgggccctctagtgaaaactcgtcctggggagtaggacagctgctgagaagcagagaggaatgcggccagctggggaaaatgggacagcaggggtcagggaggtgattggaagggcagacaccatagtccccagctacctggcttcaagagcccccgttccccacacgcctcttcttctaaggcaaggtctttccctctggggactgactgagacagcagtcactggccaggctcttggtacaaaggcaggaagggtagctctgagaacggggctttcagccgcagcactccgtgctccaggtcgatgcagcactgcggggtgtagagcagtcatgccaggtcacctcagcccgccacctgcctcccggcctgctccttttgttccccctcccacttcccacagcttccacctgccttttgctcttcccccatccccatttccctagactcctgttgaagggggtgacccagttctcttgatttttcacttggtggtaagtaaggaacctctaaggaagcaaagggacagttgcccatctctaagtcactctcatcagaacctggtccaggttccacacctgtgccttctactactttttcccagtgctttgggtcaggccctgagtgggtgccttaccttgagagaaagcagagtctgcaggcccaggcagaattcaggactctcagcatctataggaacaatttgaaaacagaagaggctgagggttcccagtggtcactgctgccctcctcttagccgttgctccttctctgcccaccccatccccagatccgaggacactggcacagagatgggggatagtcagaacatctctgggaactcctcgtgctgcagggagtgaaagtctcagcctttgccccaccccaaagagaaaggtgaggtgagcaccagggctgttgcagaaggggggacttacccaccacctgtgccgagcacaccacagtctcctgccccagctgtagctccaactgctccacctgggttgggggcccaggggccaggtccccagctgaggcttttaggacccttttctctaaccccaggcggctgagacatccagcagagatccgattgtattgggtgcctgtgtcaacggccactctaagcagctggtcctggcacttgcagttgaccagaagagctggaatctctgtcctgctggtcttcctcctgctctcctggccatgaatcaggtcctgcatccggggaggctccccctgaagccaattcgggtttccctccaccaggcgtctttggatcacactgcgcggctgcaagtccttggaggtgccgagcctcttgaggctgtccagcgggagcaggtcggccgagtccttgtgcaggaactgggtggcctgtttgagccggcgctgctggctcaggtgggctcggtctcgaagctgtgcctcctgccccctcgtcctggcttctccctcatctctcctggcctcctgcttggtgctcatggcccctgctggaggagtgggccaggggctgctcggtgggggcgtcaccgagtcctctctgcttcttcctgcctgtctctgtcccgtgctgcagctctctttccaacaggagggtctccacgggagggaaagaggaaaaataaataacatgcaggagcagccgcgtcagtctccaatttcccgagattgctgtagagggagt

SEQ ID NO: 16094 - RNA, 2076 nt, Homo sapiens
  source 1..2076: mol_type = other RNA
gctgggattacaggcatgagccattgcgcctggcctctttctttactcctaatccatgatttgagagactcaaaccagccagaaagactctcagggatctggcgtcttaaggttcgggttcttctcttcacagtgaattcaaaaaagcctctgtctcctgacagaccccaaactttaaaaaaaaaaaaaaagcctctgtctttttgctttggcaaagcctggcagggggttagaaagccactgattccaggacaatacaagcttaagctcaagaggccagagatggggataggaagaaggcctaatgaggtggatagttctagaaatcagaaagaatgctgaataggtgaagtctgagtggtgacaacctcactgtcctgtctgcctcacaggagcagttctctacaaggctcttccacacacacacacgcaaggctcaggggctcggtgggtacaaaaagccagtggaaacggataaatacctatagcgttaatagcagaagtatgtccaaggttttgcacagggtaatcaaactaactggcttcagacatttgcagccacaggaaaaaatagctctcagccttatgagatggacattcctatactaactcccgctctttgttgtattgaattctggctgtttcttcccccactcaactgtgagcagatgtgcacagactccgagaggcagacaccaggaggtccagggacataggttggtgaggcatggcggtctagttgtgggagataatgaggcccagaaggtgtggtgagagacatggtggtgtgggaagttgagttgtgtttggggtggtattgggtgatggacaaggacagcagtcagcagagccttcgacccagcccaagcaggcaccccattgtgcttaggttcctatctgtggtcttgatttggctttgcttttcttgggaggaagatgaatcagaatcctggcatcgtgggccctctagtgaaaactcgtcctggggagtaggacagctgctgagaagcagagaggaatgcggccagctggggaaaatgggacagcaggggtcagggaggtgattggaagggcagacaccatagtccccagctacctggcttcaagagcccccgttccccacacgcctcttcttctaaggcaaggtctttccctctggggactgactgagacagcagtcactggccaggctcttggtacaaaggcaggaagggtagctctgagaacggggctttcagccgcagcactccgtgctccaggtcgatgcagcacttgagagaaagcagagtctgcaggcccaggcagaattcaggactctcagcatccaccacctgtgccgagcacaccacagtctcctgccccagctgtagctccaactgctccacctgggttgggggcccaggggccaggtccccagctgaggcttttaggacccttttctctaaccccaggcggctgagacatccagcagagatccgattgtattgggtgcctgtgtcaacggccactctaagcagctggtcctggcacttgcagttgaccagaagagctggaatctctgtcctgctggtcttcctcctgctctcctggccatgaatcaggtcctgcatccggggaggctccccctgaagccaattcgggtttccctccaccaggcgtctttggatcacactgcgcggctgcaagtccttggaggtgccgagcctcttgaggctgtccagcgggagcaggtcggccgagtccttgtgcaggaactgggtggcctgtttgagccggcgctgctggctcaggtgggctcggtctcgaagctgtgcctcctgccccctcgtcctggcttctccctcatctctcctggcctcctgcttggtgctcatggcccctgctggaggagtgggccaggggctgctcggtgggggcgtcaccgagtcctctctgcttcttcctgcctgtctctgtcccgtgctgcagctctctttccaacaggagggtctccacgggagggaaagaggaaaaataaataacatgcaggagcagccgcgtcagtctccaatttcccgagattgctgtagagggagt

SEQ ID NO: 16095 - RNA, 2038 nt, Homo sapiens
  source 1..2038: mol_type = other RNA
gctgggattacaggcatgagccattgcgcctggcctctttctttactcctaatccatgatttgagagactcaaaccagccagaaagactctcagggatctggcgtcttaaggttcgggttcttctcttcacagtgaattcaaaaaagcctctgtctcctgacagaccccaaactttaaaaaaaaaaaaaaagcctctgtctttttgctttggcaaagcctggcagggggttagaaagccactgattccaggacaatacaagcttaagctcaagaggccagagatggggataggaagaaggcctaatgaggtggatagttctagaaatcagaaagaatgctgaataggtgaagtctgagtggtgacaacctcactgtcctgtctgcctcacaggagcagttctctacaaggctcttccacacacacacacgcaaggctcaggggctcggtgggtacaaaaagccagtggaaacggataaatacctatagcgttaatagcagaagtatgtccaaggttttgcacagggtaatcaaactaactggcttcagacatttgcagccacaggaaaaaatagctctcagccttatgagatggacattcctatactaactcccgctctttgttgtattgaattctggctgtttcttcccccactcaactgtgagcagatgtgcacagactccgagaggcagacaccaggaggtccagggacataggttggtgaggcatggcggtctagttgtgggagataatgaggcccagaaggtgtggtgagagacatggtggtgtgggaagttgagttgtgtttggggtggtattgggtgatggacaaggacagcagtcagcagagccttcgacccagcccaagcaggcaccccattgtgcttaggttcctatctgtggtcttgatttggctttgcttttcttgggaggaagatgaatcagaatcctggcatcgtgggccctctagtgaaaactcgtcctggggagtaggacagctgctgagaagcagagaggaatgcggccagctggggaaaatgggacagcaggggtcagggaggtgattggaagggcagacaccatagtccccagctacctggcttcaagagcccccgttccccacacgcctcttcttctaaggcaaggtctttccctctggggactgactgagacagcagtcactggccaggctcttggtacaaaggcaggaagggtagctctgagaacggggctttcagccgcagcactccgtgctccaggtcgatgcagcacttgagagaaagcagagtctgcaggcccaggcagaattcaggactctcagcatccaccacctgtgccgagcacaccacagtctcctgccccagctgtagctccaactgctccacctgggttgggggcccaggggccaggtccccagctgaggcttttaggacccttttctctaaccccaggcggctgagacatccagcagagatccgattgtattgggtgcctgtgtcaacggccactctaagcagctggtcctggcacttgcagttgaccagaagagctggaatctctgtcctgctggtcttcctcctgctctcctggccatgaatcaggtcctgcatccggggaggctccccctgaagccaattcgggtttccctccaccaggcgtctttggatcacactgcgcggctgcaagtccttggaggtgccgagcctcttgaggctgtccagcgggagcaggtcggccgagtccttgtgcaggaactgggtggcctgtttgagccggcgctgctggctcaggtgggctcggtctcgaagctgtgcctcctgccccctcgtcctggcttctccctcatctctcctggcctcctgcttggtgctcatggcccctgctggaggagtgggccaggggctgctcggtgggggcgtcaccgagtcctctctgcttcttcctgcctgtctctgtcccgtgctgcagctctctttccaacaggagggtcttgttaggtctcttgcctcccgcctagcagatgtcagagtctttaact

SEQ ID NO: 16096 - RNA, 1833 nt, Homo sapiens
  source 1..1833: mol_type = other RNA
gctgggattacaggcatgagccattgcgcctggcctctttctttactcctaatccatgatttgagagactcaaaccagccagaaagactctcagggatctggcgtcttaaggttcgggttcttctcttcacagtgaattcaaaaaagcctctgtctcctgacagaccccaaactttaaaaaaaaaaaaaaagcctctgtctttttgctttggcaaagcctggcagggggttagaaagccactgattccaggacaatacaagcttaagctcaagaggccagagatggggataggaagaaggcctaatgaggtggatagttctagaaatcagaaagaatgctgaataggtgaagtctgagtggtgacaacctcactgtcctgtctgcctcacaggagcagttctctacaaggctcttccacacacacacacgcaaggctcaggggctcggtgggtacaaaaagccagtggaaacggataaatacctatagcgttaatagcagaagtatgtccaaggttttgcacagggtaatcaaactaactggcttcagacatttgcagccacaggaaaaaatagctctcagccttatgagatggacattcctatactaactcccgctctttgttgtattgaattctggctgtttcttcccccactcaactgtgagcagatgtgcacagactccgagaggcagacaccaggaggtccagggacataggttggtgaggcatggcggtctagttgtgggagataatgaggcccagaaggtgtggtgagagacatggtggtgtgggaagttgagttgtgtttggggtggtattgggtgatggacaaggacagcagtcagcagagccttcgacccagcccaagcaggcaccccattgtgcttaggttcctatctgtggtcttgatttggctttgcttttcttgggaggaagatgaatcagaatcctggcatcgtgggccctctagtgaaaactcgtcctggggagtaggacagctgctgagaagcagagaggaatgcggccagcttgagagaaagcagagtctgcaggcccaggcagaattcaggactctcagcatccaccacctgtgccgagcacaccacagtctcctgccccagctgtagctccaactgctccacctgggttgggggcccaggggccaggtccccagctgaggcttttaggacccttttctctaaccccaggcggctgagacatccagcagagatccgattgtattgggtgcctgtgtcaacggccactctaagcagctggtcctggcacttgcagttgaccagaagagctggaatctctgtcctgctggtcttcctcctgctctcctggccatgaatcaggtcctgcatccggggaggctccccctgaagccaattcgggtttccctccaccaggcgtctttggatcacactgcgcggctgcaagtccttggaggtgccgagcctcttgaggctgtccagcgggagcaggtcggccgagtccttgtgcaggaactgggtggcctgtttgagccggcgctgctggctcaggtgggctcggtctcgaagctgtgcctcctgccccctcgtcctggcttctccctcatctctcctggcctcctgcttggtgctcatggcccctgctggaggagtgggccaggggctgctcggtgggggcgtcaccgagtcctctctgcttcttcctgcctgtctctgtcccgtgctgcagctctctttccaacaggagggtctccacgggagggaaagaggaaaaataaataacatgcaggagcagccgcgtcagtctccaatttcccgagattgctgtagagggagt

SEQ ID NO: 16097 - RNA, 1795 nt, Homo sapiens
  source 1..1795: mol_type = other RNA
gctgggattacaggcatgagccattgcgcctggcctctttctttactcctaatccatgatttgagagactcaaaccagccagaaagactctcagggatctggcgtcttaaggttcgggttcttctcttcacagtgaattcaaaaaagcctctgtctcctgacagaccccaaactttaaaaaaaaaaaaaaagcctctgtctttttgctttggcaaagcctggcagggggttagaaagccactgattccaggacaatacaagcttaagctcaagaggccagagatggggataggaagaaggcctaatgaggtggatagttctagaaatcagaaagaatgctgaataggtgaagtctgagtggtgacaacctcactgtcctgtctgcctcacaggagcagttctctacaaggctcttccacacacacacacgcaaggctcaggggctcggtgggtacaaaaagccagtggaaacggataaatacctatagcgttaatagcagaagtatgtccaaggttttgcacagggtaatcaaactaactggcttcagacatttgcagccacaggaaaaaatagctctcagccttatgagatggacattcctatactaactcccgctctttgttgtattgaattctggctgtttcttcccccactcaactgtgagcagatgtgcacagactccgagaggcagacaccaggaggtccagggacataggttggtgaggcatggcggtctagttgtgggagataatgaggcccagaaggtgtggtgagagacatggtggtgtgggaagttgagttgtgtttggggtggtattgggtgatggacaaggacagcagtcagcagagccttcgacccagcccaagcaggcaccccattgtgcttaggttcctatctgtggtcttgatttggctttgcttttcttgggaggaagatgaatcagaatcctggcatcgtgggccctctagtgaaaactcgtcctggggagtaggacagctgctgagaagcagagaggaatgcggccagcttgagagaaagcagagtctgcaggcccaggcagaattcaggactctcagcatccaccacctgtgccgagcacaccacagtctcctgccccagctgtagctccaactgctccacctgggttgggggcccaggggccaggtccccagctgaggcttttaggacccttttctctaaccccaggcggctgagacatccagcagagatccgattgtattgggtgcctgtgtcaacggccactctaagcagctggtcctggcacttgcagttgaccagaagagctggaatctctgtcctgctggtcttcctcctgctctcctggccatgaatcaggtcctgcatccggggaggctccccctgaagccaattcgggtttccctccaccaggcgtctttggatcacactgcgcggctgcaagtccttggaggtgccgagcctcttgaggctgtccagcgggagcaggtcggccgagtccttgtgcaggaactgggtggcctgtttgagccggcgctgctggctcaggtgggctcggtctcgaagctgtgcctcctgccccctcgtcctggcttctccctcatctctcctggcctcctgcttggtgctcatggcccctgctggaggagtgggccaggggctgctcggtgggggcgtcaccgagtcctctctgcttcttcctgcctgtctctgtcccgtgctgcagctctctttccaacaggagggtcttgttaggtctcttgcctcccgcctagcagatgtcagagtctttaact

SEQ ID NO: 16098 - RNA, 1956 nt, Homo sapiens
  source 1..1956: mol_type = other RNA
gctgggattacaggcatgagccattgcgcctggcctctttctttactcctaatccatgatttgagagactcaaaccagccagaaagactctcagggatctggcgtcttaaggttcgggttcttctcttcacagtgaattcaaaaaagcctctgtctcctgacagaccccaaactttaaaaaaaaaaaaaaagcctctgtctttttgctttggcaaagcctggcagggggttagaaagccactgattccaggacaatacaagcttaagctcaagaggccagagatggggataggaagaaggcctaatgaggtggatagttctagaaatcagaaagaatgctgaataggtgaagtctgagtggtgacaacctcactgtcctgtctgcctcacaggagcagttctctacaaggctcttccacacacacacacgcaaggctcaggggctcggtgggtacaaaaagccagtggaaacggataaatacctatagcgttaatagcagaagtatgtccaaggttttgcacagggtaatcaaactaactggcttcagacatttgcagccacaggaaaaaatagctctcagccttatgagatggacattcctatactaactcccgctctttgttgtattgaattctggctgtttcttcccccactcaactgtgagcagatgtgcacagactccgagaggcagacaccaggaggtccagggacataggttggtgaggcatggcggtctagttgtgggagataatgaggcccagaaggtgtggtgagagacatggtggtgtgggaagttgagttgtgtttggggtggtattgggtgatggacaaggacagcagtcagcagagccttcgacccagcccaagcaggcaccccattgtgcttaggttcctatctgtggtcttgatttggctttgcttttcttgggaggaagatgaatcagaatcctggcatcgtgggccctctagtgaaaactcgtcctggggagtaggacagctgctgagaagcagagaggaatgcggccagtgagacagcagtcactggccaggctcttggtacaaaggcaggaagggtagctctgagaacggggctttcagccgcagcactccgtgctccaggtcgatgcagcacttgagagaaagcagagtctgcaggcccaggcagaattcaggactctcagcatccaccacctgtgccgagcacaccacagtctcctgccccagctgtagctccaactgctccacctgggttgggggcccaggggccaggtccccagctgaggcttttaggacccttttctctaaccccaggcggctgagacatccagcagagatccgattgtattgggtgcctgtgtcaacggccactctaagcagctggtcctggcacttgcagttgaccagaagagctggaatctctgtcctgctggtcttcctcctgctctcctggccatgaatcaggtcctgcatccggggaggctccccctgaagccaattcgggtttccctccaccaggcgtctttggatcacactgcgcggctgcaagtccttggaggtgccgagcctcttgaggctgtccagcgggagcaggtcggccgagtccttgtgcaggaactgggtggcctgtttgagccggcgctgctggctcaggtgggctcggtctcgaagctgtgcctcctgccccctcgtcctggcttctccctcatctctcctggcctcctgcttggtgctcatggcccctgctggaggagtgggccaggggctgctcggtgggggcgtcaccgagtcctctctgcttcttcctgcctgtctctgtcccgtgctgcagctctctttccaacaggagggtctccacgggagggaaagaggaaaaataaataacatgcaggagcagccgcgtcagtctccaatttcccgagattgctgtagagggagtgagactccggctggaaaaa

SEQ ID NO: 16099 - RNA, 2597 nt, Homo sapiens
  source 1..2597: mol_type = other RNA
gctgggattacaggcatgagccattgctcccaaccatgatatggattcttgattttcccaagtttttgagccttacaccctatttaggatgtggcatggcatccagaagctccagctagcctcgtgatgctgggtcaatcttgcagcctcactgagccactttccccatgtataagcctggggagggatccctgccctggaacctacctccgattcacacacaggaaagtgctcagaagagtttcaaagcccctcatgccccagagagcattggtacccatgactgatggctccatgcctcccttccacagccatttcctgagcatctactatgaaccatgaagccaggagctggggacagccgataactcagccaggattctggccatctaggagtttaaaacttagactccaggaatcgatatcagtctccctcctcccttcctatgtaaaagataagagttaggaacttcaaacttctgacaaaggggaatgacttgattttccagagaccttgagagaatcacaagagaacgaggttttccccttaggaagagagttagaggaatggcccagttttcttcccaagcctgaaaacatgggacaaggagaagggcaggaggatgggagaaacgggtagaagtgggggcaacacacacatccaggatgaggtatgggtaagatacatcttcaggcttgtctcacacttgagagattcactgataaggaaagccaagccagaaaatcttgagtgccccttctgtgctaaagtcattcccagagatcccacagagtcaccactcaactgagcgtctatgtatgaaaagcccaaaacacaatgcttgatgatgacccagccagaaactctgaagagtttctccgctctttagctcaaggtcagctttttaacaggctgtcttctagaaggtgctagagaagagcaatttattttgaaatctggtcacacaccagattctgattttgtgttgtcttttcacaacaggcctgctgtgtttatgacttggttgagacaaacttttttttttcaaaaaaaggtatcgcatccttctgttagatgtgttgttggcaacggttgctagggagagctgggttcagttacagacacactgatgccggctctaataatactttgctctgcatagctcggatgcagacacctcttggctaaacagagcacacacatttcaacagaggagggcttgaacttgtactacccaagcctgtctcagcaaaggagcattcccagagcccacgtggacgtcccggggcagtgacagggcagtgctgggtggagagggctcaggcttccattcctgtcattccaaaggtcccataaaaagaggcacactcgttcttcacttctctgtgaaactggagccccttcaccgccctgtatcacaccacaattccctgatgaggatccaaggaaacttttggttccttctctaacccaggcaccctgggcaccccacattctcctggaagtcggaaacaatcaatgcacatcatctagttagtcagtctagtctgcagtcaggaccctgcaaagccagagaagttgggaaccttggtgggaaggtgtatggggagacaggctgaactgcgaagtgtggcccagcctctggtacagcctggcaccgtgggtgagaatgaggcccttttcctaaaacatgtgatagctgttccgacacacatcccaggccaaggaaaaggaaaatgggaaaaggagctgaggacagagagaaatggaggcagcgggagagaagaggtggctttcatctcatcaaggaggaggttcagggtgatgacaagaagagcctgaggctgggggagtggaaggcatgttctcagcagctgaggcctcctgtgtaatggggttctcctgccagctcagactcggagttttcccccatggctcagcagagagcccaacacctggcaggtatttcttgactggttcgcggcatgacaggcagagccagctgattcataagtggccgcgatgaaccagttcggtgtctctggggtgtctcctcaacagtggtgttccaccctggctaacgaatgcccaggttgcgtccttggagaatctaattcaactgattaggggtaggccccctgcctgctgtgttctcatgattctcatgcatagcgaggctgagaaccactgacctaaagaagagccagtatctgaaatgcaatattcccaggccagacctccactctgaccatcacactgatgacagactgtgccttagtttgcccatctatgaaacagagccaccacctacaaaccatcagtcattcaatgccttgtgacttcccactgtggtccctggactagagcactagcatctaccaggagcatgtttgaaacgcagaatctcaagcccatcccaggcctcttgcatcagaatctgcatttaaacaaaatcccacgtgattcatatgcacattccggtttgagaacccctgacctaataaagacaacatgcttggcacattaagaaatgtctgttttgttgtggggtggggggaggggggagggatagcattaggagatatacctaatgtta

SEQ ID NO: 16100 - RNA, 1377 nt, Homo sapiens
  source 1..1377: mol_type = other RNA
gctgggattacaggcatgagccattggcccttagggcttttgaagtaggaaagccagtggctcacatttggagttaactagttggaagagaggatctagaccccaggacccccaggtacgttctgtgtattaggtattaaacctgctttgcaaaccaggaagctggggttcaaagattaagtgacttgctcaaggtcaggcaagaagtgatagatccgggatttaaatgtgccaatctgcacctttctggcacaagctctgagattttgctattgcaggttgcaagagatgcccccattgaatggttatgtccagcccttctgtctacagcacagtgttctgaaaggcttaggagcacagaactgaaatgctggcctttctgtattcctgcctatttggctttggtgggccttttcttttttttttttttttttggagatagggtcttcttctgtcacccaggccggagtgcagtggcgtgatcacggctcactgcagcctacacctcccgggcttgagtgatctgctaccagagctgttttcttctcccagggatacttggtccttatcactcccatctagacggttacttccttttttttttgaaacggagtcttgctctgtcacccaggctggagtgcagtggtgtgttctcagctccctgcaacctccaccccaagaagctgggatcacaggcgtgcgccaccacgcccggtaaatttttgtatgtttagtaaagactgggtttcgccatgtttgccaggctggtgtcgaactcctgacctcaagtgatccacccacctcggcctcccaaaatgctgggattacaggcgagagccaccgcgacctgcttagacattctacttcgttagagccttagagcctatctcagatactttcttccaggcaccttgcgtatttctcaacttttgccgataacaacatgttattggcttgtctttttctcttacctagattatcaaccttcaagttttttgtgcatgatttgatccaccccttcccaccacatcaccacagtacctaccagtggtgatgagagctaccgttgactttgccatattttgcagagcggtgaagacactagctttggagaagtacaatggcaaggtcgcacagctttagtccagccagagaagtcttgtgagtccttaaacctaacacagacacttcttgaggtcggcttcagcatcctctcctccaggaagccaccctggtgcctggtgagtggcttcctgggatcacccatgcctcagtgtgcaggatgagagggctggtcctgatccccttctgtcctcacccccaggtccatgtccagggcttaggactggtcgtcccttggtgttgactcatctccca

SEQ ID NO: 16101 - RNA, 3182 nt, Homo sapiens
  source 1..3182: mol_type = other RNA
gctgggattacaggcatgagccattgggtctagctggccttactgattaggttttgttgctgggagggtattctatagcagctcatgctgagatttctagagagcaccaatgtcactactaactattgattcctatttatttctcatggttttatgactccttggctttagacaacaggctgtattatacctttgtgttggacttcgtcagtacctgtcattcaccctgctcatgttaagtatcatcattacaaagtgatggaatgagagaaaagcacaaagctctaaatgttggttcttggattttaacctcaatccagtaggctcataaccctctcttggttcaaagccatacaagtccacattccttgctctccaatatttaactggcacccacagagaaagtacaaacttcaaaaccacaacacaggccaacaggatagctgtgttttgtttcctctgccctgaggcacaactggatctagcaccaaggagggcaggatttaacagaccagcacaagacaaatcaatttaaagaggtagtttgaaccaggaataagactgcagtgtagactacaactgaacagaatacaaatccaatgtggttcttcactgagaacaggggttttggccacttgtaatgtaattaaacccccacgaataacaaagatgattatatggaggatgaggatctgcttggtataagcacagttgttggagcctgaggaaaacctggccatcaacaaaccacagcctgagtctttccaaagagaaagctgggcttttgcccttctggcccatgactggtagatttacactgcagatcaaaggtctctctcaacaatcaaactacttccaagaaaccatagacctttaaaaataaggactagtgatttcatacaggctagtaaaaatactttggctatagcccttcacacatgtgtgcttgggtacacatacacacaggtggagctcaataaatgtggaatgattaggtattgatcagcagtatttactacgtgagttaagtccagacacaccatctaccaatcagcaattcaaatttccatgcccaataccaggcagccaacccaccaggcaatatttccttagcttaaagcacagattctcaaaagtgtggtcccttgtaacatcagcaggaactcagaagtgccactttgggggcttttgggttgaggcccagcaattagtgttttaacaagccctacaggtgattctgatgcacgctaaagcttgaaaatcacagttttagaggcagacatgcgaaaacattataatggaaaaattaattcaaactctcttgcttcacttcagctgggacaaaccaaggtatcaagacaaagtaaactgtgaatggttttatttaaaaatatctatttctattttctcaaattgattgtcattttttgattggcaagttcatgctaatcaaagtgttaagtgggaatgcaagtcgatgcatcagccatccaagaatacacactctgcaagttctaagcctgtatttagtctcaaaccaccgctctgcacactacaaagattttggtataacgtatcacatctagagaaaggcacaatgtatttcccactcattgaatccaaaagctggaccttcttttctttttttttgagatggagtttcactcttgtcacccaggctggagtgcaatggcgccatcttggctcactgcaacctccgcctcctaggttcaagtgattctcctgcctcagccttctgagtagctgggattacaggcgcccaccaccatgcccggctaatttttgtatttttagtagagacggggtttccccatgttggccagactggtctcgaactcctgtcctcaggtgatccagcctgccttggccccccaaagtgctgggattacaggcatgggccactgtgtccggccctggaccttattttctaatgttaagtttgagttctgggtttagttgggcaagaatttccctcagctgccatcaatcctggctgaagttaacccctttccatcactgacccaggggaaaaaaccaccaaatttacttactatctgttaaaaattcaaaaaggaagcagatgatcaagtcattgaacaaaaagctacatggattagacaagaacatataacttggctctaagatgatggagaaggaaaagacatctcatgggtggcttctccttaagagaaatgggaatctcagcttattagaaaaaacaatttgggaggttactactttagttcagagactgtaaactaaacctctgttgagcaggggtgtgtgtgtgtgtgtgtgtgtgtgtgtgtgtacgtgcacaaagaggagcaagaagggatgattggagcaggaatcacgtcttcaagtcttcaacaacttcccactgcaatcgataaggccacgccatagagtttgatgtcaatggcaatgctctgtgatatccactaccactgccttcttccagctgaagaggaagtatcctgtaccggcccctgctgctactgcaatgcagaggtacccgttgtaggtcatgaagatgagcatgaggaagtagcttatgaccacctggatgatgtgcagcactgtttgcaggaggtgaggaaagctcagcatctgttgcccaacagttttgtgtgtctccataaggatggttccatttggtcctgggacaggcatggaattgtagcgaatgctgacttgtgacttacgcagcaggctctctcgggctatcttgagtccttcatagaacattgctagtaaaaacactgccacaaaagctccagccatttctccagctgtattgatcaccaaaccggaaaacagtagttccacattcttaaagccaaagtagaaggtcataggcatcatcatcatgctgctgtctcctccaccatgggagtgtgaggctgaagtggttgggtgatggtgagaaggttgcatggtactgttggagtccatatagctcatccccatatggtgggaatgatccattttttccaggaaaagttgagagtcagcagaagattctttccaggtcaagtccagccactagcacctctctctccgaatcttaacccgtcaccccctcacgactcttcgaacggcccctccacttctacccggctcgacgtgtccaccaccgccaccgaggccgaggattt

SEQ ID NO: 16102 - RNA, 3295 nt, Homo sapiens
  source 1..3295: mol_type = other RNA
gctgggattacaggcatgagccattgtgcccagcctatatagtgtgaagcttttaggaaaatcagaacagggtagacagctgttaaaaacaatgtttaaatggaataatgttgaatgtttacaggctgtaagaactattgtatacacaaaataatacacaaagtttgtactttgtgtacaaatacaaatttgtactttgtgtacaaataatacaaaaagtttgtatacacaaactttttacgttgtggtttggtatattgtcttaactgaattttcttataagaaccccatgaaacttacctgagtttttaaaatgctatccaggacatcataccttatagtatacatgaaacataatgtaatccaggttgtaatttagaactttttttttttttttagctgagcacttaatgtaattaattccaggttatgactcttaaaaaacattggccattagagaaatagttctatttgcccatccaaatcacctgaatgactttttgaaagaataggggtccacatccccagatcccatcccagctgtgcacagtctgaagcaagcagagtgaaacaagttggcaacttgttccaagcgtgggcctttgcagtctgtgatccagtgttactccaggtcccagtctgtcccatacttgtcttttgctacagttagttagttactttgttatcatccccttgtaaactgccttcaatatcgtgtttgaaaggaaaaaaaataaatccatagtaactaatggtctgccgattttttccctgaatttttaaactccaacaaagcattattttgcaaaaagtcctttagcccaaagtcagtgtctctgttttgatctctttgtaaaagaactctctgttcatccattctctttccctgggaccgtaaaataaggctgaaaaagtcttcatctggtactgtcggaccctttgtggtagcaggtggtggagcacatctttgatcatctaatctggatccttgacattttacaaggatgtcaaagaaatcttcatcagcctctttgttgtcattagtcatcaggtggctaagtaccgactggctgttttgtgttagacgaagccctggcaaattactgaaactagccctctggtcatccagacggcgactctgtgagctggcaagaagatctaaaaactcatccgtgttgggggataccacaggaacagatgatgtttttagcatcattttagggggagtggaagaagttgttgttgaagctgtatggcagttcttttcttgtaagcaacatctctgatcatccatcctattgctttgaaatcggcttaataagtcaaagaacccttcatctccaatagtatctgcactgattttcctctgagaatttggaattcggtggtcaatagaattactggcatcttggagaactttagtggaggaattcgttttgtattttttccccttcagtctgttgacaaagagtagctttgcagaaggtttggcaataagaggtttttgcttagcaagaatttcactgttccagttctgtaccttttctggtgttaacttcataagttccatattttccatactatgccggcgtcccaacttggggcgtacaccattcaaactgctatcaatttcagtattttcagacattatggagttatttgtgctgtagctcagaccaagaaccatttgaaggtctgagagattaagtcgtgctgttagttcaccacttttatccccaacctctcttgaaatttccaagtgcttttcagcaaaatgcattgcttgatcatgatttcctagtgctgtgtatgcatttcctaagctccaacatgctcttccttcaccaattctatcattcagctcttgagcaattgctaagtgcttcagatgataatcaatggccttttcatagtcttgaagtaaagtatatgtatttccaagactgtaacaagactgtgcttctacagctcggtctttaagctgtcgggccaacagtagtgtcttcttgtagtattccgaggcagtttcaaattcaccaagaaatatatatgcatttccaaggttgctatatgctcttctttcagctgctttatctccaaattcttttgcaataaggagacgctgctcatgagctataactgcatccctgaagttgccaaggaggtaatgtgtgtttccaagatttccaaaggcacgtccttgtgccgctcggtcacccaaagcagtcactaatgataggttttcctcataaaaatccacggctgcctgcagagcatctctcacttcttctggaaattctcctacatcctggggaccagggcaaccaaaacttttccctttggcatgatacacattcccaagattgtaaagtgctcttgcttctcccaccttgtcattaagctctctggaaatatctaggtgtcgctgacaacaaactatggcttcgtcaaaattcccaagaacttttaaggtgtttcccagattaccactagctttcgcttcccccagctggtctccaatagtccttgcaagggttaaatcatgatggtgatattctaatgctttggcataatcatgcaaatagaaataagcattgcccaactggctgtaaatagcgctaagtgtttttaggtcttcagttccaacttgaactgcagcttcaaagaatgacacgccagcgcggcagtctcctgatttacatagacgttccccttccaaggccagctctaggcaagaagcttccattctgtaacgaacatgaaaagaatggtcttctctcatgcttatcaaattttcctccatcgagtcatattataagctgaataaaataaaattattttattttgtgccaatccagtcctttacaatgtagaattgtttgtagaacattgtccggttagtatattaatgagttggtgttaatacatcctaagctcctgattcttctttattaataatgaaaggaggtcaatgtcagacagcttaaaggttcaaaatgtatcccaaatccttgcatctctggccctttcagcagcacttcagcaacatttctcccgcgggcgggcgggtcccgggtacgcggtgaaggtgcagcggcggccgcctcgggcgacagacgggtggtcacggcccctccccaaggcaggggcaccgcaggaggccggcgcgccccctgctcccgcccccggcaggtcacgtgggccagagctcgtagcgcccctcgctttcccggagcgtccctccgccacctaggggtcccgccgctccgccggtctcaacaccgccctcctctgc

SEQ ID NO: 16103 - RNA, 4400 nt, Homo sapiens
  source 1..4400: mol_type = other RNA
gctgggattacaggcatgagccattgtgcccagcctatatagtgtgaagcttttaggaaaatcagaacagggtagacagctgttaaaaacaatgtttaaatggaataatgttgaatgtttacaggctgtaagaactattgtatacacaaaataatacacaaagtttgtactttgtgtacaaatacaaatttgtactttgtgtacaaataatacaaaaagtttgtatacacaaactttttacgttgtggtttggtatattgtcttaactgaattttcttataagaaccccatgaaacttacctgagtttttaaaatgctatccaggacatcataccttatagtatacatgaaacataatgtaatccaggttgtaatttagaactttttttttttttttagctgagcacttaatgtaattaattccaggttatgactcttaaaaaacattggccattagagaaatagttctatttgcccatccaaatcacctgaatgactttttgaaagaataggggtccacatccccagatcccatcccagctgtgcacagtctgaagcaagcagagtgaaacaagttggcaacttgttccaagcgtgggcctttgcagtctgtgatccagtgttactccaggtcccagtctgtcccatacttgtcttttgctacagttagttagttactttgttatcatccccttgtaaactgccttcaatatctgggataaggaagacaaagcttaatgacaactaaggttctagctgacatctttctttcatatttaatttttgtgagttttcatctgttttctgtttgtttatgtgtcctaggttcttgacctaaccacatgggttttgttttttgtttttatattagaacttagaaaagtttgttttacagcagtattatggaacagaagagaccattttaaataatttttttaaacagcccaaaacacacaaaagatacttgttttctagagacagggtcttgctctgtcacccaggctggagtgcagtggcacgatcatagctcagtgcagcctccacctcctgggctcaagtggtcctcctgcctcagcctcttaagcagttgggactacaggtgtgtgccagcatgcttgctgttttttttttttttgagacagagtcttgctctgtcactcaggctggagtccagtggcttggtctcagctcactgcaatctctgcctcccaggggttcaagtgattctcctgcctcagcctcccaagtagctgaaactacaggcgcatgccaccatgcccagctaatttttgtatttttagtagagacagggtttcactatgttggccaggctggtctcaaactcccgacctcaagtgatccgcccgcttcggcctcccaaagtgctgggattacaggtgtgagccactgcgcctggctgctgatttatttttcatagacacgggggtctatgttgcccaggttggtcttgaactcctagcctcaagcgatcctcctgcctcagcctcccaatgtgctgggattacaggaatgagccaccatgcccagcccaagaagtagagtttcttttatactgactttggcctaaaaaaacagattttcatggaggaaaaaaaaacctagatttttagtaagactattttatatacttttttacattgatcaagtacattatttttaccaaacaacattgtttcccactacatccatggttatgtataaaaaaacgccattgtcaattaagatgttaaaaaattatttccataagagtattaaattctaatctatgattcacttaacttcctactttataaacactaggtaaagtaatctcacaagctgccaaagaacacatcccaagcagtaatcacagacgatgaagcaccttacaggacccctccaccctcaaacgcgcatgtccagagaagtattaatgccttaatagactactgaaggttaactatttacatcattctaaaaatattttaagctgtattacagtgctataaattctccttttaaggaaaaaagtaatagattgtttccttaccgtgtttgaaaggaaaaaaaataaatccatagtaactaatggtctgccgattttttccctgaatttttaaactccaacaaagcattattttgcaaaaagtcctttagcccaaagtcagtgtctctgttttgatctctttgtaaaagaactctctgttcatccattctctttccctgggaccgtaaaataaggctgaaaaagtcttcatctggtactgtcggaccctttgtggtagcaggtggtggagcacatctttgatcatctaatctggatccttgacattttacaaggatgtcaaagaaatcttcatcagcctctttgttgtcattagtcatcaggtggctaagtaccgactggctgttttgtgttagacgaagccctggcaaattactgaaactagccctctggtcatccagacggcgactctgtgagctggcaagaagatctaaaaactcatccgtgttgggggataccacaggaacagatgatgtttttagcatcattttagggggagtggaagaagttgttgttgaagctgtatggcagttcttttcttgtaagcaacatctctgatcatccatcctattgctttgaaatcggcttaataagtcaaagaacccttcatctccaatagtatctgcactgattttcctctgagaatttggaattcggtggtcaatagaattactggcatcttggagaactttagtggaggaattcgttttgtattttttccccttcagtctgttgacaaagagtagctttgcagaaggtttggcaataagaggtttttgcttagcaagaatttcactgttccagttctgtaccttttctggtgttaacttcataagttccatattttccatactatgccggcgtcccaacttggggcgtacaccattcaaactgctatcaatttcagtattttcagacattatggagttatttgtgctgtagctcagaccaagaaccatttgaaggtctgagagattaagtcgtgctgttagttcaccacttttatccccaacctctcttgaaatttccaagtgcttttcagcaaaatgcattgcttgatcatgatttcctagtgctgtgtatgcatttcctaagctccaacatgctcttccttcaccaattctatcattcagctcttgagcaattgctaagtgcttcagatgataatcaatggccttttcatagtcttgaagtaaagtatatgtatttccaagactgtaacaagactgtgcttctacagctcggtctttaagctgtcgggccaacagtagtgtcttcttgtagtattccgaggcagtttcaaattcaccaagaaatatatatgcatttccaaggttgctatatgctcttctttcagctgctttatctccaaattcttttgcaataaggagacgctgctcatgagctataactgcatccctgaagttgccaaggaggtaatgtgtgtttccaagatttccaaaggcacgtccttgtgccgctcggtcacccaaagcagtcactaatgataggttttcctcataaaaatccacggctgcctgcagagcatctctcacttcttctggaaattctcctacatcctggggaccagggcaaccaaaacttttccctttggcatgatacacattcccaagattgtaaagtgctcttgcttctcccaccttgtcattaagctctctggaaatatctaggtgtcgctgacaacaaactatggcttcgtcaaaattcccaagaacttttaaggtgtttcccagattaccactagctttcgcttcccccagctggtctccaatagtccttgcaagggttaaatcatgatggtgatattctaatgctttggcataatcatgcaaatagaaataagcattgcccaactggctgtaaatagcgctaagtgtttttaggtcttcagttccaacttgaactgcagcttcaaagaatgacacgccagcgcggcagtctcctgatttacatagacgttccccttccaaggccagctctaggcaagaagcttccattctgtaacgaacatgaaaagaatggtcttctctcatgcttatcaaattttcctccatcgagtcatattataagctcccgcgggcgggcgggtcccgggtacgcggtgaaggtgcagcggcggccgcctcgggcgacagacgggtggtcacggcccctccccaaggcaggggcaccgcaggaggccggcgcgccccctgctcccgcccccggcaggtcacgtgggccagagctcgtagcgcccctcgctttcccggagcgtccctccgccacctaggggtcccgccgctccgccggtctcaacaccgccctcctctgc

SEQ ID NO: 16104 - RNA, 4632 nt, Homo sapiens
  source 1..4632: mol_type = other RNA
gctgggattacaggcatgagccattgtgcccagcctatatagtgtgaagcttttaggaaaatcagaacagggtagacagctgttaaaaacaatgtttaaatggaataatgttgaatgtttacaggctgtaagaactattgtatacacaaaataatacacaaagtttgtactttgtgtacaaatacaaatttgtactttgtgtacaaataatacaaaaagtttgtatacacaaactttttacgttgtggtttggtatattgtcttaactgaattttcttataagaaccccatgaaacttacctgagtttttaaaatgctatccaggacatcataccttatagtatacatgaaacataatgtaatccaggttgtaatttagaactttttttttttttttagctgagcacttaatgtaattaattccaggttatgactcttaaaaaacattggccattagagaaatagttctatttgcccatccaaatcacctgaatgactttttgaaagaataggggtccacatccccagatcccatcccagctgtgcacagtctgaagcaagcagagtgaaacaagttggcaacttgttccaagcgtgggcctttgcagtctgtgatccagtgttactccaggtcccagtctgtcccatacttgtcttttgctacagttagttagttactttgttatcatccccttgtaaactgccttcaatatctgggataaggaagacaaagcttaatgacaactaaggttctagctgacatctttctttcatatttaatttttgtgagttttcatctgttttctgtttgtttatgtgtcctaggttcttgacctaaccacatgggttttgttttttgtttttatattagaacttagaaaagtttgttttacagcagtattatggaacagaagagaccattttaaataatttttttaaacagcccaaaacacacaaaagatacttgttttctagagacagggtcttgctctgtcacccaggctggagtgcagtggcacgatcatagctcagtgcagcctccacctcctgggctcaagtggtcctcctgcctcagcctcttaagcagttgggactacaggtgtgtgccagcatgcttgctgttttttttttttttgagacagagtcttgctctgtcactcaggctggagtccagtggcttggtctcagctcactgcaatctctgcctcccaggggttcaagtgattctcctgcctcagcctcccaagtagctgaaactacaggcgcatgccaccatgcccagctaatttttgtatttttagtagagacagggtttcactatgttggccaggctggtctcaaactcccgacctcaagtgatccgcccgcttcggcctcccaaagtgctgggattacaggtgtgagccactgcgcctggctgctgatttatttttcatagacacgggggtctatgttgcccaggttggtcttgaactcctagcctcaagcgatcctcctgcctcagcctcccaatgtgctgggattacaggaatgagccaccatgcccagcccaagaagtagagtttcttttatactgactttggcctaaaaaaacagattttcatggaggaaaaaaaaacctagatttttagtaagactattttatatacttttttacattgatcaagtacattatttttaccaaacaacattgtttcccactacatccatggttatgtataaaaaaacgccattgtcaattaagatgttaaaaaattatttccataagagtattaaattctaatctatgattcacttaacttcctactttataaacactaggtaaagtaatctcacaagctgccaaagaacacatcccaagcagtaatcacagacgatgaagcaccttacaggacccctccaccctcaaacgcgcatgtccagagaagtattaatgccttaatagactactgaaggttaactatttacatcattctaaaaatattttaagctgtattacagtgctataaattctccttttaaggaaaaaagtaatagattgtttccttaccgtgtttgaaaggaaaaaaaataaatccatagtaactaatggtctgccgattttttccctgaatttttaaactccaacaaagcattattttgcaaaaagtcctttagcccaaagtcagtgtctctgttttgatctctttgtaaaagaactctctgttcatccattctctttccctgggaccgtaaaataaggctgaaaaagtcttcatctggtactgtcggaccctttgtggtagcaggtggtggagcacatctttgatcatctaatctggatccttgacattttacaaggatgtcaaagaaatcttcatcagcctctttgttgtcattagtcatcaggtggctaagtaccgactggctgttttgtgttagacgaagccctggcaaattactgaaactagccctctggtcatccagacggcgactctgtgagctggcaagaagatctaaaaactcatccgtgttgggggataccacaggaacagatgatgtttttagcatcattttagggggagtggaagaagttgttgttgaagctgtatggcagttcttttcttgtaagcaacatctctgatcatccatcctattgctttgaaatcggcttaataagtcaaagaacccttcatctccaatagtatctgcactgattttcctctgagaatttggaattcggtggtcaatagaattactggcatcttggagaactttagtggaggaattcgttttgtattttttccccttcagtctgttgacaaagagtagctttgcagaaggtttggcaataagaggtttttgcttagcaagaatttcactgttccagttctgtaccttttctggtgttaacttcataagttccatattttccatactatgccggcgtcccaacttggggcgtacaccattcaaactgctatcaatttcagtattttcagacattatggagttatttgtgctgtagctcagaccaagaaccatttgaaggtctgagagattaagtcgtgctgttagttcaccacttttatccccaacctctcttgaaatttccaagtgcttttcagcaaaatgcattgcttgatcatgatttcctagtgctgtgtatgcatttcctaagctccaacatgctcttccttcaccaattctatcattcagctcttgagcaattgctaagtgcttcagatgataatcaatggccttttcatagtcttgaagtaaagtatatgtatttccaagactgtaacaagactgtgcttctacagctcggtctttaagctgtcgggccaacagtagtgtcttcttgtagtattccgaggcagtttcaaattcaccaagaaatatatatgcatttccaaggttgctatatgctcttctttcagctgctttatctccaaattcttttgcaataaggagacgctgctcatgagctataactgcatccctgaagttgccaaggaggtaatgtgtgtttccaagatttccaaaggcacgtccttgtgccgctcggtcacccaaagcagtcactaatgataggttttcctcataaaaatccacggctgcctgcagagcatctctcacttcttctggaaattctcctacatcctggggaccagggcaaccaaaacttttccctttggcatgatacacattcccaagattgtaaagtgctcttgcttctcccaccttgtcattaagctctctggaaatatctaggtgtcgctgacaacaaactatggcttcgtcaaaattcccaagaacttttaaggtgtttcccagattaccactagctttcgcttcccccagctggtctccaatagtccttgcaagggttaaatcatgatggtgatattctaatgctttggcataatcatgcaaatagaaataagcattgcccaactggctgtaaatagcgctaagtgtttttaggtcttcagttccaacttgaactgcagcttcaaagaatgacacgccagcgcggcagtctcctgatttacatagacgttccccttccaaggccagctctaggcaagaagcttccattctgtaacgaacatgaaaagaatggtcttctctcatgcttatcaaattttcctccatcgagtcatattataagctgaataaaataaaattattttattttgtgccaatccagtcctttacaatgtagaattgtttgtagaacattgtccggttagtatattaatgagttggtgttaatacatcctaagctcctgattcttctttattaataatgaaaggaggtcaatgtcagacagcttaaaggttcaaaatgtatcccaaatccttgcatctctggccctttcagcagcacttcagcaacatttctcccgcgggcgggcgggtcccgggtacgcggtgaaggtgcagcggcggccgcctcgggcgacagacgggtggtcacggcccctccccaaggcaggggcaccgcaggaggccggcgcgccccctgctcccgcccccggcaggtcacgtgggccagagctcgtagcgcccctcgctttcccggagcgtccctccgccacctaggggtcccgccgctccgccggtctcaacaccgccctcctctgc

SEQ ID NO: 16105 - RNA, 899 nt, Homo sapiens
  source 1..899: mol_type = other RNA
gctgggattacaggcatgagccattgtgcccggctattccttccctcttcacccaagttgggggctcggaggggctgcagagttggcacttgtggacatcttcagaccctggcattactgaaggagctgttgccctgtgtgcgtcctatagcatttctgtccctatgtctcaatactgtatttttatctgtgtgtgcacgcactctgtgtgtgtgagagaatgtgtgtgtgtgtgtgtgtgagagagagagagagagaggtgtgtgtgtgtgtgtgtgtgtgtgtgtcagggttctccgtttgtgtctgttttagtccagggtagccttttgtgtgtgcctttatgccaagtgctccagatggtgatttacaggggtaaaatgacccctggtggccaaatcagagaactgacccagattcctcagggatagccatgaaatctgggcctttctccatctgggtggagattggagcctggagcccggcacttacctccagccgctctggaagaggcctggtgattagcacctgctccatctctcttcatcttcagggttcaagacctgtgcccttcctgtcctgagagcactggcagcgccaaacctcgtagtccaaaatcttagcactttgcccatgttgtccttgccagaggagcacggaaagtcctggaaggtgaactttctcactcagggtttggggaatcccaaaggctccagaaccagacagagctctgccagcaatcagacgtaggaccacgggaggtggtgagcaaggcaggctgggcaggtttccacggtgctaggtcaagcaggcagtctttaggggcagcgactggcctgttgccctctgggggcactctctccccactaggcccatgtccatcccacagaccaaggagg

SEQ ID NO: 16106 - RNA, 3916 nt, Homo sapiens
  source 1..3916: mol_type = other RNA
gctgggattacaggcatgagccattgtgcctggctgactacctcttaaggaaacttttttgtttagttagacaaagaatggtaaatctctttccacgcacattcaaaattcacacattatctggactcttagttacctaggacatacccccagttattcttgtacctaatttggtacctcaaattttcccgaggtgttaaaacaaaaggaatagagcttgcctagcaccttagaagtgctgcaccctcttagaagtgccaggcactgtcatagttgttgccctcttagaatgatttgcctctgggtgtcactctttgctctgtacctggtacaactatagtgatggcagatgctccatactcagtcctagcttttcagtgtttggctttgctgggttttttctttctttctttttgagagaaatggggacttccaagctgagtaaaacctggaaagggcaacttactgcagccatatattgatactacattatttcctatgtcataatattaacctcccttccatctgcttttgctgtttagtagtctcatgtcttcttgagctagactatcttatgtaaattcatgttatgtgaattgaggtctcagtaataacagccttctgtctttcctcaccgtaacaggagtcataggaaagggggtgtgatagtctcagaaacagcctagcatctcatacaaacttgtttctgtttttgagacagggtctcgctctatcacccaggctggagtgcagtggcacaatcatggctcactgcagccttgatctcctgggctcctgtctcagcctcccaagtagctgggactacgtgcatgcatgcaccactacacctagctttttttttcttttttcttttttcttgtaatagagataggatctcactttgttgcccaggctggtctcaaactgggctcaagttatcttcccaccttggcctcccaaagtgctgggattataggcatgagccaccacattcagcccaaacatttctgagaccactacttgaactatcaagtctcctcttgtaactgattctcattagaaataatacacatttattgaatgtcattgatatataaagataccattctttgagtgggggaaatataatttaaaagtcgcaactactgacaatcaacaaataaactctaatgagaatcataaagcttgttcccagagaaccatgatacagggtgggacagtacgcaaataatgggctcctgttgtcagacttcatggtgattacattagtgctttctccagtatctttcttcctattgtactcctgaagcactcagaatgataaagataaatttctgatcattcctacaaagagtgcaggcaaagttaagatttaactgtgattgctggttgtttcatctcgaattcaaaatcctggatttccgaaacaatggagcttgatgtcacatttggctatcttgcttttgtctcctcttctggaaagaacaaatcatcttcctgaaaattacaggagacacttagtatgacaaaataaggcctctgaaactgtccaatctcacatgtaaaaagtgtaaaatcacagaactaaaatcaggttccggattttcctggaaatagaatgtcaccgggatctgttcaaaggtgagctttggctacattttataacagtgtttaaaactcgaatgcaaaaaactgctttcaatataatcagatatgtgcaaaaacaatttgttaaataacatgggaagattatattaacaaaagacatttccagaatactaacattcatgtgatttataaaggtgcattttctgtaaagagctatacagcccaaaaacatgaaattcttcaagggagtcccctttatcccatgagttggaagaatttattttcatattctatgcatggatcactgaagtgatgaatgtcactcgtcttcaagaaggaagcactctcagccttgtgaagaagaacctcaagggttcctggggctatgatcatgaagagcaccacaatgaagactgctgcgaagtctttttcacttcttcacatttgggatgtgaaatattttacagaaaaataagagtgtgcaaatccctctcacacatagaaaaacgattgtgtgaatattcttaaatttttaaaacttttaaaaactgtgatctttgcactgttttcaagagtcagcaactctgaagaaagatattcaccataagtgaccccatatggtgaagatattcacaataaatgacagttttgcaagatgactctttgggttggcattctgtttccggtcaccaggtttccgcaatctctgtgacagcccgcagcagctcggcaaatgtagggcggccttcaggtttctcatgccagcagctgtacatgacttcatatatggacattggtgccaggtgagggcgatatagcctgaagccttcagaaatagcttccacgacttgcaaatttgacttattttcaaaaggcatttttccttctgtaaaaacttcccacattaaaactccaaatgaccagacatcagatttactgctgtacttattgaaaagaaaaacttcaggaggggaccacttgattgggaacttggctccaaaagaactgacatactcatcatccaaaacgtaccttgtcattccaaagtctgaaatttttactatgcatgttgaactgaccaaacaattccttgccgccaaatccctatgaatatagccattcctctccagatattccattccttcacatatatcctggcatacactcagtagcatttccttcctaagctttcctttattctccctgagatagttaagcaggcagccattttccatgaactctgtcacaatgtaaaggggcttccgctgtatacagactccataaagttgcactagctttgaatgagataatttcatcatcactttggcctcttcaatgaaatcctcttcagacatggagccttcattgatggccttgatagctacctggatatgtgaccgccattcacctaaatggaccactccaaactgaccgcttccaatctcctttataaaagccaactcagatggatctatctcccacttttcgtagctaaacccagctgtggctggtaaacaactgcccatcagcccaactggatatcggagacgagtcatgagaccggctgcattgtgctggtgataccagattaactcagggattgattgaaaggcgtgtctttcagccacataccactgtcctgagtcattcttttttatctgataatgttttatggcagcctccgtacttcttctagctcccataaatacggaaattgtgtaggatcctaaatgtcttgaatctctgacaataaatgcaccttctttagactcttgtctcaatagatgttctgcctgatttctggtaatgtttctatggtaccaccccaaacggtctcttgccttccaccagtgaggattgtatttctccagtatcaggtattcttctgctctccttaaggctaaattacagggttctctgggcagaaaatcataaagtgccttgacttggatcttctcttcagcaacctcagagggtgggaggggaggcagtggctttcgttttgacggctgcacacggcccgtgttggattgcttcttatttgacaattggctgagccacggcctgcgacgctgggtgtatttttctggaagctcttcatctgtgctcaggcttatctgtgttctcatttgtctcatttgatggtgtctttttgttataaatagacatggtatagtgattaggaacaagagtttgaatcccagctccaccatttcatagtgtggccttgggtaagcaatgtaacctctctaatcttcaatttcctcatcgcttctgcactgaacagcaacagcagcaacagaaaacc

SEQ ID NO: 16107 - RNA, 4975 nt, Homo sapiens
  source 1..4975: mol_type = other RNA
gctgggattacaggcatgagccattgtgcctggctgactacctcttaaggaaacttttttgtttagttagacaaagaatggtaaatctctttccacgcacattcaaaattcacacattatctggactcttagttacctaggacatacccccagttattcttgtacctaatttggtacctcaaattttcccgaggtgttaaaacaaaaggaatagagcttgcctagcaccttagaagtgctgcaccctcttagaagtgccaggcactgtcatagttgttgccctcttagaatgatttgcctctgggtgtcactctttgctctgtacctggtacaactatagtgatggcagatgctccatactcagtcctagcttttcagtgtttggctttgctgggttttttctttctttctttttgagagaaatggggacttccaagctgagtaaaacctggaaagggcaacttactgcagccatatattgatactacattatttcctatgtcataatattaacctcccttccatctgcttttgctgtttagtagtctcatgtcttcttgagctagactatcttatgtaaattcatgttatgtgaattgaggtctcagtaataacagccttctgtctttcctcaccgtaacaggagtcataggaaagggggtgtgatagtctcagaaacagcctagcatctcatacaaacttgtttctgtttttgagacagggtctcgctctatcacccaggctggagtgcagtggcacaatcatggctcactgcagccttgatctcctgggctcctgtctcagcctcccaagtagctgggactacgtgcatgcatgcaccactacacctagctttttttttcttttttcttttttcttgtaatagagataggatctcactttgttgcccaggctggtctcaaactgggctcaagttatcttcccaccttggcctcccaaagtgctgggattataggcatgagccaccacattcagcccaaacatttctgagaccactacttgaactatcaagtctcctcttgtaactgattctcattagaaataatacacatttattgaatgtcattgatatataaagataccattctttgagtgggggaaatataatttaaaagtcgcaactactgacaatcaacaaataaactctaatgagaatcataaagcttgttcccagagaaccatgatacagggtgggacagtacgcaaataatgggctcctgttgtcagacttcatggtgattacattagtgctttctccagtatctttcttcctattgtactcctgaagcactcagaatgataaagataaatttctgatcattcctacaaagagtgcaggcaaagttaagatttaactgtgattgctggttgtttcatctcgaattcaaaatcctggatttccgaaacaatggagcttgatgtcacatttggctatcttgcttttgtctcctcttctggaaagaacaaatcatcttcctgaaaattacaggagacacttagtatgacaaaataaggcctctgaaactgtccaatctcacatgtaaaaagtgtaaaatcacagaactaaaatcaggttccggattttcctggaaatagaatgtcaccgggatctgttcaaaggtgagctttggctacattttataacagtgtttaaaactcgaatgcaaaaaactgctttcaatataatcagatatgtgcaaaaacaatttgttaaataacatgggaagattatattaacaaaagacatttccagaatactaacattcatgtgatttataaaggtgcattttctgtaaagagctatacagcccaaaaacatgaaattcttcaagggagtcccctttatcccatgagttggaagaatttattttcatattctatgcatggatcactgaagtgatgaatgtcactcgtcttcaagaaggaagcactctcagccttgtgaagaagaacctcaagggttcctggggctatgatcatgaagagcaccacaatgaagactgctgcgaagtctttttcacttcttcacatttgggatgtgaaatattttacagaaaaataagagtgtgcaaatccctctcacacatagaaaaacgattgtgtgaatattcttaaatttttaaaacttttaaaaactgtgatctttgcactgttttcaagagtcagcaactctgaagaaagatattcaccataagtgaccccatatggtgaagatattcacaataaatgacagttttgcaagatgactctttgggttggcattctgtttccggtcaccaggtttccgcaatctctgtgacagcccgcagcagctcggcaaatgtagggcggccttcaggtttctcatgccagcagctgtacatgacttcatatatggacattggtgccaggtgagggcgatatagcctgaagccttcagaaatagcttccacgacttgcaaatttgacttattttcaaaaggcatttttccttctgtaaaaacttcccacattaaaactccaaatgaccagacatcagatttactgctgtacttattgaaaagaaaaacttcaggaggggaccacttgattgggaacttggctccaaaagaactgacatactcatcatccaaaacgtaccttgtcattccaaagtctgaaatttttactatgcatgttgaactgaccaaacaattccttgccgccaaatccctatgaatatagccattcctctccagatattccattccttcacatatatcctggcatacactcagtagcatttccttcctaagctttcctttattctccctgagatagttaagcaggcagccattttccatgaactctgtcacaatgtaaaggggcttccgctgtatacagactccataaagttgcactagctttgaatgagataatttcatcatcactttggcctcttcaatgaaatcctcttcagacatggagccttcattgatggccttgatagctacctggatatgtgaccgccattcacctaaatggaccactccaaactgaccgcttccaatctcctttataaaagccaactcagatggatctatctcccacttttcgtagctaaacccagctgtggctggtaaacaactgcccatcagcccaactggatatcggagacgagtcatgagaccggctgcattgtgctggtgataccagattaactcagggattgattgaaaggcgtgtctttcagccacataccactgtcctgagtcattcttttttatctgataatgttttatggcagcctccgtacttcttctagctcccataaatacggaaattgtgtaggatcctaaatgtcttgaatctctgacaataaatgcaccttctttagactcttgtctcaatagatgttctgcctgatttctggtaatgtttctatggtaccactcatatatttctaaattagttattttgttttcagtcacatagttgcttgggattaagccttcattccccaaacggtctcttgccttccaccagtgaggattgtatttctccagtatcaggtattcttctgctctccttaaggctaaattacagggttctctgggcagaaaatcataaagtgccttgacttggatcttctcttcagcaacctcagagggtgggaggggaggcagtggctttcgttttgacggctgcacacggcccgtgttggattgcttcttatttgacaattggctgagccacggcctgcgacgctgggtgtatttttctggaagctcttcatctgtgctcaggcttatctgtgttctcatttgtaggaggaaaggatcatggtagccccttctgcggggagcacacaacagtcttcagttcttctgcggtgctctactcacaaaaacacatctttcaactgaaatcatagttcgctcaagatgtttctcacgggcagagttaaccccacctattttcctgttctgaaaacctcagaagagtataaatgacaaccaatggcatatataagaaagctcagtaatctccatcccaatctctgagggtatctgctattagtctctcatccccaaaggtgtgggtgactcgcaaacatcattttcaagaaatcacaaaattttggtaaaaggcacctttaaaattatcaaatcaaactgccctctctggactgggaaggaaatgaaggcacagacagaataagggacttgcccaaggccacaccgtgagtggcagaaacaattagattctaggctctggaatattgagtttagaatgttccatcctcccactcagcagacactttatttgggggaagtcaatctagtaataaccctaaaatgtgattgggggatggctgagaaatataaaaacaccaacaatacaaaacacacttgggagtttcacttcatcccactggaaagcataaccatgtgtcaactaattaacagagcaactttaatgaagacacagcatattctaatcgcccttccaatttcctggtttagattaaggtctccttagcattctgggtgatgactgttatttttacttcaccttttgcctttgttatgctttcgtataaaactttttttctaagtcttagtgaaaaatatttaaagatttttgaaggaaatgttgacaaatgttgccaggtgctatctatcttgttttcccataaaaagcatacactgaccattaggacagggactctatcttctcctcactctctttcataccacctagtacttcccgtagctcctcaaggtgaaaagggaagtatgggatgggaggagggaaggtcaggaaggaaggagaaaaggctgacagtgatagtaaggtagagtgtgccaggaccgactccttcaatgagctacaagtcagttaaaagttgtgcatggttagcaaccaaaatgcccatcaatgataggctggataaagaaaatgtggtacatatacaccgtggaatattatgcag

SEQ ID NO: 16108 - RNA, 3981 nt, Homo sapiens
  source 1..3981: mol_type = other RNA
gctgggattacaggcatgagccattgtgcctggctgactacctcttaaggaaacttttttgtttagttagacaaagaatggtaaatctctttccacgcacattcaaaattcacacattatctggactcttagttacctaggacatacccccagttattcttgtacctaatttggtacctcaaattttcccgaggtgttaaaacaaaaggaatagagcttgcctagcaccttagaagtgctgcaccctcttagaagtgccaggcactgtcatagttgttgccctcttagaatgatttgcctctgggtgtcactctttgctctgtacctggtacaactatagtgatggcagatgctccatactcagtcctagcttttcagtgtttggctttgctgggttttttctttctttctttttgagagaaatggggacttccaagctgagtaaaacctggaaagggcaacttactgcagccatatattgatactacattatttcctatgtcataatattaacctcccttccatctgcttttgctgtttagtagtctcatgtcttcttgagctagactatcttatgtaaattcatgttatgtgaattgaggtctcagtaataacagccttctgtctttcctcaccgtaacaggagtcataggaaagggggtgtgatagtctcagaaacagcctagcatctcatacaaacttgtttctgtttttgagacagggtctcgctctatcacccaggctggagtgcagtggcacaatcatggctcactgcagccttgatctcctgggctcctgtctcagcctcccaagtagctgggactacgtgcatgcatgcaccactacacctagctttttttttcttttttcttttttcttgtaatagagataggatctcactttgttgcccaggctggtctcaaactgggctcaagttatcttcccaccttggcctcccaaagtgctgggattataggcatgagccaccacattcagcccaaacatttctgagaccactacttgaactatcaagtctcctcttgtaactgattctcattagaaataatacacatttattgaatgtcattgatatataaagataccattctttgagtgggggaaatataatttaaaagtcgcaactactgacaatcaacaaataaactctaatgagaatcataaagcttgttcccagagaaccatgatacagggtgggacagtacgcaaataatgggctcctgttgtcagacttcatggtgattacattagtgctttctccagtatctttcttcctattgtactcctgaagcactcagaatgataaagataaatttctgatcattcctacaaagagtgcaggcaaagttaagatttaactgtgattgctggttgtttcatctcgaattcaaaatcctggatttccgaaacaatggagcttgatgtcacatttggctatcttgcttttgtctcctcttctggaaagaacaaatcatcttcctgaaaattacaggagacacttagtatgacaaaataaggcctctgaaactgtccaatctcacatgtaaaaagtgtaaaatcacagaactaaaatcaggttccggattttcctggaaatagaatgtcaccgggatctgttcaaaggtgagctttggctacattttataacagtgtttaaaactcgaatgcaaaaaactgctttcaatataatcagatatgtgcaaaaacaatttgttaaataacatgggaagattatattaacaaaagacatttccagaatactaacattcatgtgatttataaaggtgcattttctgtaaagagctatacagcccaaaaacatgaaattcttcaagggagtcccctttatcccatgagttggaagaatttattttcatattctatgcatggatcactgaagtgatgaatgtcactcgtcttcaagaaggaagcactctcagccttgtgaagaagaacctcaagggttcctggggctatgatcatgaagagcaccacaatgaagactgctgcgaagtctttttcacttcttcacatttgggatgtgaaatattttacagaaaaataagagtgtgcaaatccctctcacacatagaaaaacgattgtgtgaatattcttaaatttttaaaacttttaaaaactgtgatctttgcactgttttcaagagtcagcaactctgaagaaagatattcaccataagtgaccccatatggtgaagatattcacaataaatgacagttttgcaagatgactctttgggttggcattctgtttccggtcaccaggtttccgcaatctctgtgacagcccgcagcagctcggcaaatgtagggcggccttcaggtttctcatgccagcagctgtacatgacttcatatatggacattggtgccaggtgagggcgatatagcctgaagccttcagaaatagcttccacgacttgcaaatttgacttattttcaaaaggcatttttccttctgtaaaaacttcccacattaaaactccaaatgaccagacatcagatttactgctgtacttattgaaaagaaaaacttcaggaggggaccacttgattgggaacttggctccaaaagaactgacatactcatcatccaaaacgtaccttgtcattccaaagtctgaaatttttactatgcatgttgaactgaccaaacaattccttgccgccaaatccctatgaatatagccattcctctccagatattccattccttcacatatatcctggcatacactcagtagcatttccttcctaagctttcctttattctccctgagatagttaagcaggcagccattttccatgaactctgtcacaatgtaaaggggcttccgctgtatacagactccataaagttgcactagctttgaatgagataatttcatcatcactttggcctcttcaatgaaatcctcttcagacatggagccttcattgatggccttgatagctacctggatatgtgaccgccattcacctaaatggaccactccaaactgaccgcttccaatctcctttataaaagccaactcagatggatctatctcccacttttcgtagctaaacccagctgtggctggtaaacaactgcccatcagcccaactggatatcggagacgagtcatgagaccggctgcattgtgctggtgataccagattaactcagggattgattgaaaggcgtgtctttcagccacataccactgtcctgagtcattcttttttatctgataatgttttatggcagcctccgtacttcttctagctcccataaatacggaaattgtgtaggatcctaaatgtcttgaatctctgacaataaatgcaccttctttagactcttgtctcaatagatgttctgcctgatttctggtaatgtttctatggtaccactcatatatttctaaattagttattttgttttcagtcacatagttgcttgggattaagccttcattccccaaacggtctcttgccttccaccagtgaggattgtatttctccagtatcaggtattcttctgctctccttaaggctaaattacagggttctctgggcagaaaatcataaagtgccttgacttggatcttctcttcagcaacctcagagggtgggaggggaggcagtggctttcgttttgacggctgcacacggcccgtgttggattgcttcttatttgacaattggctgagccacggcctgcgacgctgggtgtatttttctggaagctcttcatctgtgctcaggcttatctgtgttctcatttgtctcatttgatggtgtctttttgttataaatagacatggtatagtgattaggaacaagagtttgaatcccagctccaccatttcatagtgtggccttgggtaagcaatgtaacctctctaatcttcaatttcctcatcgcttctgcactgaacagcaacagcagcaacagaaaac

SEQ ID NO: 16109 - RNA, 3399 nt, Homo sapiens
  source 1..3399: mol_type = other RNA
gctgggattacaggcatgagccattgtgcctggctgactacctcttaaggaaacttttttgtttagttagacaaagaatggtaaatctctttccacgcacattcaaaattcacacattatctggactcttagttacctaggacatacccccagttattcttgtacctaatttggtacctcaaattttcccgaggtgttaaaacaaaaggaatagagcttgcctagcaccttagaagtgctgcaccctcttagaagtgccaggcactgtcatagttgttgccctcttagaatgatttgcctctgggtgtcactctttgctctgtacctggtacaactatagtgatggcagatgctccatactcagtcctagcttttcagtgtttggctttgctgggttttttctttctttctttttgagagaaatggggacttccaagctgagtaaaacctggaaagggcaacttactgcagccatatattgatactacattatttcctatgtcataatattaacctcccttccatctgcttttgctgtttagtagtctcatgtcttcttgagctagactatcttatgtaaattcatgttatgtgaattgaggtctcagtaataacagccttctgtctttcctcaccgtaacaggagtcataggaaagggggtgtgatagtctcagaaacagcctagcatctcatacaaacttgtttctgtttttgagacagggtctcgctctatcacccaggctggagtgcagtggcacaatcatggctcactgcagccttgatctcctgggctcctgtctcagcctcccaagtagctgggactacgtgcatgcatgcaccactacacctagctttttttttcttttttcttttttcttgtaatagagataggatctcactttgttgcccaggctggtctcaaactgggctcaagttatcttcccaccttggcctcccaaagtgctgggattataggcatgagccaccacattcagcccaaacatttctgagaccactacttgaactatcaagtctcctcttgtaactgattctcattagaaataatacacatttattgaatgtcattgatatataaagataccattctttgagtgggggaaatataatttaaaagtcgcaactactgacaatcaacaaataaactctaatgagaatcataaagcttgttcccagagaaccatgatacagggtgggacagtacgcaaataatgggctcctgttgtcagacttcatggtgattacattagtgctttctccagtatctttcttcctattgtactcctgaagcactcagaatgataaagataaatttctgatcattcctacaaagagtgcaggcaaagttaagatttaactgtgattgctggttgtttcatctcgaattcaaaatcctggatttccgaaacaatggagcttgatgtcacatttggctatcttgcttttgtctcctcttctggaaagaacaaatcatcttcctgaaaattacaggagacacttagtatgacaaaataaggcctctgaaactgtccaatctcacatgtaaaaagtgtaaaatcacagaactaaaatcaggttccggattttcctggaaatagaatgtcaccgggatctgttcaaaggtgagctttggctacattttataacagtgtttaaaactcgaatgcaaaaaactgctttcaatataatcagatatgtgcaaaaacaatttgttaaataacatgggaagattatattaacaaaagacatttccagaatactaacattcatgtgatttataaaggtgcattttctgtaaagagctatacagcccaaaaacatgaaattcttcaagggagtcccctttatcccatgagttggaagaatttattttcatattctatgcatggatcactgaagtgatgaatgtcactcgtcttcaagaaggaagcactctcagccttgtgaagaagaacctcaagggttcctggggctatgatcatgaagagcaccacaatgaagactgctgcgaagtctttttcacttcttcacatttgggatgtgaaatattttacagaaaaataagagtgtgcaaatccctctcacacatagaaaaacgattgtgtgaatattcttaaatttttaaaacttttaaaaactgtgatctttgcactgttttcaagagtcagcaactctgaagaaagatattcaccataagtgaccccatatggtgaagatattcacaataaatgacagttttgcaagatgactctttgggttggcattctgtttccggtcaccaggtttccgcaatctctgtgacagcccgcagcagctcggcaaatgtagggcggccttcaggtttctcatgccagcagctgtacatgacttcatatatggacattggtgccaggtgagggcgatatagcctgaagccttcagaaatagcttccacgacttgcaaatttgacttattttcaaaaggcatttttccttctgtaaaaacttcccacattaaaactccaaatgaccagacatcagatttactgctgtacttattgaaaagaaaaacttcaggaggggaccacttgattgggaacttggctccaaaagaactgacatactcatcatccaaaacgtaccttgtcattccaaagtctgaaatttttactatgcatgttgaactgaccaaacaattccttgccgccaaatccctatgaatatagccattcctctccagatattccattccttcacatatatcctggcatacactcagtagcatttccttcctaagctttcctttattctccctgagatagttaagcaggcagccattttccatgaactctgtcacaatgtaaaggggcttccgctgtatacagactccataaagttgcactagctttgaatgagataatttcatcatcactttggcctcttcaatgaaatcctcttcagacatggagccttcattgatggccttgatagctacctggatatgtgaccgccattcacctaaatggaccactccaaactgaccgcttccaatctcctttataaaagccaactcagatggatctatctcccacttttcgtagctaaacccagctgtggctggtaaacaactgcccatcagcccaactggatatcggagacgagtcatgagaccggctgcattgtgctggtgataccagattaactcagggattgattgaaaggcgtgtctttcagccacataccactgtcctgagtcattcttttttatctgataatgttttatggcagcctccgtacttcttctagctcccataaatacggaaattgtgtaggatcctaaatgtcttgaatctctgacaataaatgcaccttctttagactgtagtcccagctactcagag

SEQ ID NO: 16110 - RNA, 3252 nt, Homo sapiens
  source 1..3252: mol_type = other RNA
gctgggattacaggcatgagccattgtgcctggctgactacctcttaaggaaacttttttgtttagttagacaaagaatggtaaatctctttccacgcacattcaaaattcacacattatctggactcttagttacctaggacatacccccagttattcttgtacctaatttggtacctcaaattttcccgaggtgttaaaacaaaaggaatagagcttgcctagcaccttagaagtgctgcaccctcttagaagtgccaggcactgtcatagttgttgccctcttagaatgatttgcctctgggtgtcactctttgctctgtacctggtacaactatagtgatggcagatgctccatactcagtcctagcttttcagtgtttggctttgctgggttttttctttctttctttttgagagaaatggggacttccaagctgagtaaaacctggaaagggcaacttactgcagccatatattgatactacattatttcctatgtcataatattaacctcccttccatctgcttttgctgtttagtagtctcatgtcttcttgagctagactatcttatgtaaattcatgttatgtgaattgaggtctcagtaataacagccttctgtctttcctcaccgtaacaggagtcataggaaagggggtgtgatagtctcagaaacagcctagcatctcatacaaacttgtttctgtttttgagacagggtctcgctctatcacccaggctggagtgcagtggcacaatcatggctcactgcagccttgatctcctgggctcctgtctcagcctcccaagtagctgggactacgtgcatgcatgcaccactacacctagctttttttttcttttttcttttttcttgtaatagagataggatctcactttgttgcccaggctggtctcaaactgggctcaagttatcttcccaccttggcctcccaaagtgctgggattataggcatgagccaccacattcagcccaaacatttctgagaccactacttgaactatcaagtctcctcttgtaactgattctcattagaaataatacacatttattgaatgtcattgatatataaagataccattctttgagtgggggaaatataatttaaaagtcgcaactactgacaatcaacaaataaactctaatgagaatcataaagcttgttcccagagaaccatgatacagggtgggacagtacgcaaataatgggctcctgttgtcagacttcatggtgattacattagtgctttctccagtatctttcttcctattgtactcctgaagcactcagaatgataaagataaatttctgatcattcctacaaagagtgcaggcaaagttaagatttaactgtgattgctggttgtttcatctcgaattcaaaatcctggatttccgaaacaatggagcttgatgtcacatttggctatcttgcttttgtctcctcttctggaaagaacaaatcatcttcctgaaaattacaggagacacttagtatgacaaaataaggcctctgaaactgtccaatctcacatgtaaaaagtgtaaaatcacagaactaaaatcaggttccggattttcctggaaatagaatgtcaccgggatctgttcaaaggtgagctttggctacattttataacagtgtttaaaactcgaatgcaaaaaactgctttcaatataatcagatatgtgcaaaaacaatttgttaaataacatgggaagattatattaacaaaagacatttccagaatactaacattcatgtgatttataaaggtgcattttctgtaaagagctatacagcccaaaaacatgaaattcttcaagggagtcccctttatcccatgagttggaagaatttattttcatattctatgcatggatcactgaagtgatgaatgtcactcgtcttcaagaaggaagcactctcagccttgtgaagaagaacctcaagggttcctggggctatgatcatgaagagcaccacaatgaagactgctgcgaagtctttttcacttcttcacatttgggatgtgaaatattttacagaaaaataagagtgtgcaaatccctctcacacatagaaaaacgattgtgtgaatattcttaaatttttaaaacttttaaaaactgtgatctttgcactgttttcaagagtcagcaactctgaagaaagatattcaccataagtgaccccatatggtgaagatattcacaataaatgacagttttgcaagatgactctttgggttggcattctgtttccggtcaccaggtttccgcaatctctgtgacagcccgcagcagctcggcaaatgtagggcggccttcaggtttctcatgccagcagctgtacatgacttcatatatggacattggtgccaggtgagggcgatatagcctgaagccttcagaaatagcttccacgacttgcaaatttgacttattttcaaaaggcatttttccttctgtaaaaacttcccacattaaaactccaaatgaccagacatcagatttactgctgtacttattgaaaagaaaaacttcaggaggggaccacttgattgggaacttggctccaaaagaactgacatactcatcatccaaaacgtaccttgtcattccaaagtctgaaatttttactatgcatgttgaactgaccaaacaattccttgccgccaaatccctatgaatatagccattcctctccagatattccattccttcacatatatcctggcatacactcagtagcatttccttcctaagctttcctttattctccctgagatagttaagcaggcagccattttccatgaactctgtcacaatgtaaaggggcttccgctgtatacagactccataaagttgcactagctttgaatgagataatttcatcatcactttggcctcttcaatgaaatcctcttcagacatggagccttcattgatggccttgatagctacctggatatgtgaccgccattcacctaaatggaccactccaaactgaccgcttccaatctcctttataaaagccaactcagatggatctatctcccacttttcgtagctaaacccagctgtggctggtaaacaactgcccatcagcccaactggatatcggagacgagtcatgagaccttctagctcccataaatacggaaattgtgtaggatcctaaatgtcttgaatctctgacaataaatgcaccttctttagactg

SEQ ID NO: 16111 - RNA, 3869 nt, Homo sapiens
  source 1..3869: mol_type = other RNA
gctgggattacaggcatgagccattgtgcctggctgactacctcttaaggaaacttttttgtttagttagacaaagaatggtaaatctctttccacgcacattcaaaattcacacattatctggactcttagttacctaggacatacccccagttattcttgtacctaatttggtacctcaaattttcccgaggtgttaaaacaaaaggaatagagcttgcctagcaccttagaagtgctgcaccctcttagaagtgccaggcactgtcatagttgttgccctcttagaatgatttgcctctgggtgtcactctttgctctgtacctggtacaactatagtgatggcagatgctccatactcagtcctagcttttcagtgtttggctttgctgggttttttctttctttctttttgagagaaatggggacttccaagctgagtaaaacctggaaagggcaacttactgcagccatatattgatactacattatttcctatgtcataatattaacctcccttccatctgcttttgctgtttagtagtctcatgtcttcttgagctagactatcttatgtaaattcatgttatgtgaattgaggtctcagtaataacagccttctgtctttcctcaccgtaacaggagtcataggaaagggggtgtgatagtctcagaaacagcctagcatctcatacaaacttgtttctgtttttgagacagggtctcgctctatcacccaggctggagtgcagtggcacaatcatggctcactgcagccttgatctcctgggctcctgtctcagcctcccaagtagctgggactacgtgcatgcatgcaccactacacctagctttttttttcttttttcttttttcttgtaatagagataggatctcactttgttgcccaggctggtctcaaactgggctcaagttatcttcccaccttggcctcccaaagtgctgggattataggcatgagccaccacattcagcccaaacatttctgagaccactacttgaactatcaagtctcctcttgtaactgattctcattagaaataatacacatttattgaatgtcattgatatataaagataccattctttgagtgggggaaatataatttaaaagtcgcaactactgacaatcaacaaataaactctaatgagaatcataaagcttgttcccagagaaccatgatacagggtgggacagtacgcaaataatgggctcctgttgtcagacttcatggtgattacattagtgctttctccagtatctttcttcctattgtactcctgaagcactcagaatgataaagataaatttctgatcattcctacaaagagtgcaggcaaagttaagatttaactgtgattgctggttgtttcatctcgaattcaaaatcctggatttccgaaacaatggagcttgatgtcacatttggctatcttgcttttgtctcctcttctggaaagaacaaatcatcttcctgaaaattacaggagacacttagtatgacaaaataaggcctctgaaactgtccaatctcacatgtaaaaagtgtaaaatcacagaactaaaatcaggttccggattttcctggaaatagaatgtcaccgggatctgttcaaaggtgagctttggctacattttataacagtgtttaaaactcgaatgcaaaaaactgctttcaatataatcagatatgtgcaaaaacaatttgttaaataacatgggaagattatattaacaaaagacatttccagaatactaacattcatgtgatttataaaggtgcattttctgtaaagagctatacagcccaaaaacatgaaattcttcaagggagtcccctttatcccatgagttggaagaatttattttcatattctatgcatggatcactgaagtgatgaatgtcactcgtcttcaagaaggaagcactctcagccttgtgaagaagaacctcaagggttcctggggctatgatcatgaagagcaccacaatgaagactgctgcgaagtctttttcacttcttcacatttgggatgtgaaatattttacagaaaaataagagtgtgcaaatccctctcacacatagaaaaacgattgtgtgaatattcttaaatttttaaaacttttaaaaactgtgatctttgcactgttttcaagagtcagcaactctgaagaaagatattcaccataagtgaccccatatggtgaagatattcacaataaatgacagttttgcaagatgactctttgggttggcattctgtttccggtcaccaggtttccgcaatctctgtgacagcccgcagcagctcggcaaatgtagggcggccttcaggtttctcatgccagcagctgtacatgacttcatatatggacattggtgccaggtgagggcgatatagcctgaagccttcagaaatagcttccacgacttgcaaatttgacttattttcaaaaggcatttttccttctgtaaaaacttcccacattaaaactccttgtcattccaaagtctgaaatttttactatgcatgttgaactgaccaaacaattccttgccgccaaatccctatgaatatagccattcctctccagatattccattccttcacatatatcctggcatacactcagtagcatttccttcctaagctttcctttattctccctgagatagttaagcaggcagccattttccatgaactctgtcacaatgtaaaggggcttccgctgtatacagactccataaagttgcactagctttgaatgagataatttcatcatcactttggcctcttcaatgaaatcctcttcagacatggagccttcattgatggccttgatagctacctggatatgtgaccgccattcacctaaatggaccactccaaactgaccgcttccaatctcctttataaaagccaactcagatggatctatctcccacttttcgtagctaaacccagctgtggctggtaaacaactgcccatcagcccaactggatatcggagacgagtcatgagaccggctgcattgtgctggtgataccagattaactcagggattgattgaaaggcgtgtctttcagccacataccactgtcctgagtcattcttttttatctgataatgttttatggcagcctccgtacttcttctagctcccataaatacggaaattgtgtaggatcctaaatgtcttgaatctctgacaataaatgcaccttctttagactcttgtctcaatagatgttctgcctgatttctggtaatgtttctatggtaccactcatatatttctaaattagttattttgttttcagtcacatagttgcttgggattaagccttcattccccaaacggtctcttgccttccaccagtgaggattgtatttctccagtatcaggtattcttctgctctccttaaggctaaattacagggttctctgggcagaaaatcataaagtgccttgacttggatcttctcttcagcaacctcagagggtgggaggggaggcagtggctttcgttttgacggctgcacacggcccgtgttggattgcttcttatttgacaattggctgagccacggcctgcgacgctgggtgtatttttctggaagctcttcatctgtgctcaggcttatctgtgttctcatttgtctcatttgatggtgtctttttgttataaatagacatggtatagtgattaggaacaagagtttgaatcccagctccaccatttcatagtgtggccttgggtaagcaatgtaacctctctaatcttcaatttcctcatcgcttctgcactgaacagcaacagcagcaacagaaaaccgactgg

SEQ ID NO: 16112 - RNA, 2935 nt, Homo sapiens
  source 1..2935: mol_type = other RNA
gctgggattacaggcatgagccattgtgctcagccctaaaatagttttgaagaatatttatacataggaaaaaatgctattttttatgcattataataattttgtaaataagaaatgtacgtgcaacaaatctacaaatatagtaaaatatagtgatgatctctctcaaaaaattgtgggaaagttgattttatattttttcctgaattgttggtgttttctacaataatgttttaaaattacagaaggcaaaagaaggcaaattcttaagatgtaaaatactcttaactcaaactacaaaacttcttcagtatcttacactaaattgaacctaaattaaacttacagttcattcaatcacagaatgtaaactccatgaaggtaacttgatttttcctgcttaatatactgttgtgcctctaatggctacatcagtacctggcacctgagtacttgttcaatgaaaggtgaagagaaaaatgaactggcagtgtatttccatcatactagcaagatgtttatttaaaaacatttaaaaactgttttttaaaaaacattctagttaagacgagataattcaatgttcaagctaataattctataccattttaagagtctgaatttacttttaagtaaaaaaaggcagagaaaaagagtgaaggatacagaattatcttgattatgcactgctgttactattcccatgctaaagaccccttttgtttcaataaaactatcaatatttactgagaatgacagctctgaatcaaaggcaagagaaagagacctgtaaatagtgctgttcatactagttgcccccagtagttcccaggcctcacttccaagctgccttaagtaatttttactttctgaatataaagccaactgtggaggggtcagacagctgaggactgaacttcttaaaaattggcttcagagaaaagcataacattacaactgaggcggccaagcacagtggctcacgtctgtaatctcagcactttgggaggctgacgcaggtggatcaccagatcaggagatagagaccatcctggctaacacagtgaaccccatctctactaaaaatacaaaaattacccgggcatggtggcatgcacctgcagtgccagctactcgggaggctgaggcaggagaattgcttgaacccgggaggcggacgttgcagtgagcagagatcgcgccactgcactccagcctgggtgacagagcaggacaccgtctcagaaaaaaaaaaaaaagttacaactgaggcatcaggtcttaaggtttaaaacagtctcataattgtcacattatcatattatgtcaactctgaaaataaatgcacactcatcccagagtctccaaaatctttatctttagaatccaaccttgttttaagaagtagtaaaatgaaggagcattgttagtagtcacctgacaaaagctgtccattattcttgacattaaaaattgaatgcaatgatttaaaaaacataatacattaacatttacataatatatttagaatcacatggtttccagtgattagatttcagtcatgcctggaaaggagaagacagtggctaggagcacattccttataaaggatacataaatggtatacttaggatgactaatattaagaatttaaacacggtgcatttttttcctcaaaggaagcaattttagtttctaaagagcatttacttctgacatctcgattcctgatttcagtggctgcagactgtgtacttctgtgccacacttaggacaagtaaagtacacgtcaaataagaaactactcttagcacagaaataacagaaaatatgctcacatcctatggtgtgaggcatggtgggccactctccacatagagcgcattctttgccactggtggctaatgtattgtcactattaggtgcaccagtaagaggaatacaccatgaagacagcttggctttcaacttctggacattgataagtggtaagagaaaaatcagaaattcagcaaaaccatgccagagaagttccctattcatgtattcaaagccaacttcacatatgttttgaggcttgcaaaatacagaatgaatacctaggagacgttctgtcaaagttgcaaactttcccctctgaaggaaaatcaaaaaattaatcagcccacctaatttcaaaagtccaatcacaaaattcacacactgcttgactttcccaaatgatgctaaatgatggtttcgaaacaaatcatagcatcgttcttctaaccacctgccaccaattgtacaaacagcataccagattttttgatttttactgggtggctgatatctcaggttaggggaaaaatcatttttgtacttaatattcaaaactgactgtcccactgtggcatttttggagtagatggtgaatctccacaagaaaacccataagcacgctttcacctctggctcaaagcgagctaacagcccaggtttaaatccatgaaagcactgagtaaactgggaccaaactagctgctccagggccttgtttagttcaagtgcatccaactggcttattcttagcactctgtttgcactcttcgcattctcttttctggaagccatgtcttctctgaaggtctcttaggagtctgcgaaacgcccacgctccacgtaactttctctgaaacattctctggaaagcttgtcttttcctagccgaatctggattaccaaggcttccggaactcgcaggcttccggagcgacgcaggagccggaagtggcaggcagtgacatgtagccgttgaggatcgccactgccttctcgttctgtggtatgaatggcagtgtctctctagagagttagtgcttaagtttgaatgatggcaggcacttcaggattccagcacgtagtagggtttaagaacgtcttagttcttacctcc

SEQ ID NO: 16113 - RNA, 2861 nt, Homo sapiens
  source 1..2861: mol_type = other RNA
gctgggattacaggcatgagccattgtgctcagccctaaaatagttttgaagaatatttatacataggaaaaaatgctattttttatgcattataataattttgtaaataagaaatgtacgtgcaacaaatctacaaatatagtaaaatatagtgatgatctctctcaaaaaattgtgggaaagttgattttatattttttcctgaattgttggtgttttctacaataatgttttaaaattacagaaggcaaaagaaggcaaattcttaagatgtaaaatactcttaactcaaactacaaaacttcttcagtatcttacactaaattgaacctaaattaaacttacagttcattcaatcacagaatgtaaactccatgaaggtaacttgatttttcctgcttaatatactgttgtgcctctaatggctacatcagtacctggcacctgagtacttgttcaatgaaaggtgaagagaaaaatgaactggcagtgtatttccatcatactagcaagatgtttatttaaaaacatttaaaaactgttttttaaaaaacattctagttaagacgagataattcaatgttcaagctaataattctataccattttaagagtctgaatttacttttaagtaaaaaaaggcagagaaaaagagtgaaggatacagaattatcttgattatgcactgctgttactattcccatgctaaagaccccttttgtttcaataaaactatcaatatttactgagaatgacagctctgaatcaaaggcaagagaaagagacctgtaaatagtgctgttcatactagttgcccccagtagttcccaggcctcacttccaagctgccttaagtaatttttactttctgaatataaagccaactgtggaggggtcagacagctgaggactgaacttcttaaaaattggcttcagagaaaagcataacattacaactgaggcggccaagcacagtggctcacgtctgtaatctcagcactttgggaggctgacgcaggtggatcaccagatcaggagatagagaccatcctggctaacacagtgaaccccatctctactaaaaatacaaaaattacccgggcatggtggcatgcacctgcagtgccagctactcgggaggctgaggcaggagaattgcttgaacccgggaggcggacgttgcagtgagcagagatcgcgccactgcactccagcctgggtgacagagcaggacaccgtctcagaaaaaaaaaaaaaagttacaactgaggcatcaggtcttaaggtttaaaacagtctcataattgtcacattatcatattatgtcaactctgaaaataaatgcacactcatcccagagtctccaaaatctttatctttagaatccaaccttgttttaagaagtagtaaaatgaaggagcattgttagtagtcacctgacaaaagctgtccattattcttgacattaaaaattgaatgcaatgatttaaaaaacataatacattaacatttacataatatatttagaatcacatggtttccagtgattagatttcagtcatgcctggaaaggagaagacagtggctaggagcacattccttataaaggatacataaatggtatacttaggatgactaatattaagaatttaaacacggtgcatttttttcctcaaaggaagcaattttagtttctaaagagcatttacttctgacatctcgattcctgatttcagtggctgcagactgtgtacttctgtgccacacttaggacaagtaaagtacacgtcaaataagaaactactcttagcacagaaataacagaaaatatgctcacatcctatggtgtgaggcatggtgggccactctccacatagagcgcattctttgccactggtggctaatgtattgtcactattaggtgcaccagtaagaggaatacaccatgaagacagcttggctttcaacttctggacattgataagtggtaagagaaaaatcagaaattcagcaaaaccatgccagagaagttccctattcatgtattcaaagccaacttcacatatgttttgaggcttgcaaaatacagaatgaatacctaggagacgttctgtcaaagttgcaaactttcccctctgaaggaaaatcaaaaaattaatcagcccacctaatttcaaaagtccaatcacaaaattcacacactgcttgactttcccaaatgatgctaaatgatggtttcgaaacaaatcatagcatcgttcttctaaccacctgccaccaattgtacaaacagcataccagattttttgatttttactgggtggctgatatctcaggttaggggaaaaatcatttttgtacttaatattcaaaactgactgtcccactgtggcatttttggagtagatggtgaatctccacaagaaaacccataagcacgctttcacctctggctcaaagcgagctaacagcccaggtttaaatccatgaaagcactgagtaaactgggaccaaactagctgctccagggccttgtttagttcaagtgcatccaactggcttattcttagcactctgtttgcactcttcgcattctcttttctggaagccatgtcttctctgaaggtctctttttcctgttcctgcagctccctcaagactggacagcctatagctatgacagtgggaatttttgctccaagttcttctgtgaaatccttgcctcatacttgccagaagctcagagacactgcaggttaggttccagaccacttaggagtctgcgaaacgcccacgctccacgtaactttctctgaaacattctctggaaagcttgtcttttcctagccgaatctggatt

SEQ ID NO: 16114 - RNA, 3077 nt, Homo sapiens
  source 1..3077: mol_type = other RNA
gctgggattacaggcatgagccattgtgctcagccctaaaatagttttgaagaatatttatacataggaaaaaatgctattttttatgcattataataattttgtaaataagaaatgtacgtgcaacaaatctacaaatatagtaaaatatagtgatgatctctctcaaaaaattgtgggaaagttgattttatattttttcctgaattgttggtgttttctacaataatgttttaaaattacagaaggcaaaagaaggcaaattcttaagatgtaaaatactcttaactcaaactacaaaacttcttcagtatcttacactaaattgaacctaaattaaacttacagttcattcaatcacagaatgtaaactccatgaaggtaacttgatttttcctgcttaatatactgttgtgcctctaatggctacatcagtacctggcacctgagtacttgttcaatgaaaggtgaagagaaaaatgaactggcagtgtatttccatcatactagcaagatgtttatttaaaaacatttaaaaactgttttttaaaaaacattctagttaagacgagataattcaatgttcaagctaataattctataccattttaagagtctgaatttacttttaagtaaaaaaaggcagagaaaaagagtgaaggatacagaattatcttgattatgcactgctgttactattcccatgctaaagaccccttttgtttcaataaaactatcaatatttactgagaatgacagctctgaatcaaaggcaagagaaagagacctgtaaatagtgctgttcatactagttgcccccagtagttcccaggcctcacttccaagctgccttaagtaatttttactttctgaatataaagccaactgtggaggggtcagacagctgaggactgaacttcttaaaaattggcttcagagaaaagcataacattacaactgaggcggccaagcacagtggctcacgtctgtaatctcagcactttgggaggctgacgcaggtggatcaccagatcaggagatagagaccatcctggctaacacagtgaaccccatctctactaaaaatacaaaaattacccgggcatggtggcatgcacctgcagtgccagctactcgggaggctgaggcaggagaattgcttgaacccgggaggcggacgttgcagtgagcagagatcgcgccactgcactccagcctgggtgacagagcaggacaccgtctcagaaaaaaaaaaaaaagttacaactgaggcatcaggtcttaaggtttaaaacagtctcataattgtcacattatcatattatgtcaactctgaaaataaatgcacactcatcccagagtctccaaaatctttatctttagaatccaaccttgttttaagaagtagtaaaatgaaggagcattgttagtagtcacctgacaaaagctgtccattattcttgacattaaaaattgaatgcaatgatttaaaaaacataatacattaacatttacataatatatttagaatcacatggtttccagtgattagatttcagtcatgcctggaaaggagaagacagtggctaggagcacattccttataaaggatacataaatggtatacttaggatgactaatattaagaatttaaacacggtgcatttttttcctcaaaggaagcaattttagtttctaaagagcatttacttctgacatctcgattcctgatttcagtggctgcagactgtgtacttctgtgccacacttaggacaagtaaagtacacgtcaaataagaaactactcttagcacagaaataacagaaaatatgctcacatcctatggtgtgaggcatggtgggccactctccacatagagcgcattctttgccactggtggctaatgtattgtcactattaggtgcaccagtaagaggaatacaccatgaagacagcttggctttcaacttctggacattgataagtggtaagagaaaaatcagaaattcagcaaaaccatgccagagaagttccctattcatgtattcaaagccaacttcacatatgttttgaggcttgcaaaatacagaatgaatacctaggagacgttctgtcaaagttgcaaactttcccctctgaaggaaaatcaaaaaattaatcagcccacctaatttcaaaagtccaatcacaaaattcacacactgcttgactttcccaaatgatgctaaatgatggtttcgaaacaaatcatagcatcgttcttctaaccacctgccaccaattgtacaaacagcataccagattttttgatttttactgggtggctgatatctcaggttaggggaaaaatcatttttgtacttaatattcaaaactgactgtcccactgtggcatttttggagtagatggtgaatctccacaagaaaacccataagcacgctttcacctctggctcaaagcgagctaacagcccaggtttaaatccatgaaagcactgagtaaactgggaccaaactagctgctccagggccttgtttagttcaagtgcatccaactggcttattcttagcactctgtttgcactcttcgcattctcttttctggaagccatgtcttctctgaaggtctctttttcctgttcctgcagctccctcaagactggacagcctatagctatgacagtgggaatttttgctccaagttcttctgtgaaatccttgcctcatacttgccagaagctcagagacactgcaggttaggttccagaccacttaggagtctgcgaaacgcccacgctccacgtaactttctctgaaacattctctggaaagcttgtcttttcctagccgaatctggattaccaaggcttccggaactcgcaggcttccggagcgacgcaggagccggaagtggcaggcagtgacatgtagccgttgaggatcgccactgccttctcgttctgtggtatgaatggcagtgtctctctagagagttagtgcttaagtttgaatgatggcaggcacttcaggattccagcacgtagtagggtttaagaacgtcttagttcttacctcc

SEQ ID NO: 16115 - RNA, 2829 nt, Homo sapiens
  source 1..2829: mol_type = other RNA
gctgggattacaggcatgagccattgtgctcagccctaaaatagttttgaagaatatttatacataggaaaaaatgctattttttatgcattataataattttgtaaataagaaatgtacgtgcaacaaatctacaaatatagtaaaatatagtgatgatctctctcaaaaaattgtgggaaagttgattttatattttttcctgaattgttggtgttttctacaataatgttttaaaattacagaaggcaaaagaaggcaaattcttaagatgtaaaatactcttaactcaaactacaaaacttcttcagtatcttacactaaattgaacctaaattaaacttacagttcattcaatcacagaatgtaaactccatgaaggtaacttgatttttcctgcttaatatactgttgtgcctctaatggctacatcagtacctggcacctgagtacttgttcaatgaaaggtgaagagaaaaatgaactggcagtgtatttccatcatactagcaagatgtttatttaaaaacatttaaaaactgttttttaaaaaacattctagttaagacgagataattcaatgttcaagctaataattctataccattttaagagtctgaatttacttttaagtaaaaaaaggcagagaaaaagagtgaaggatacagaattatcttgattatgcactgctgttactattcccatgctaaagaccccttttgtttcaataaaactatcaatatttactgagaatgacagctctgaatcaaaggcaagagaaagagacctgtaaatagtgctgttcatactagttgcccccagtagttcccaggcctcacttccaagctgccttaagtaatttttactttctgaatataaagccaactgtggaggggtcagacagctgaggactgaacttcttaaaaattggcttcagagaaaagcataacattacaactgaggcggccaagcacagtggctcacgtctgtaatctcagcactttgggaggctgacgcaggtggatcaccagatcaggagatagagaccatcctggctaacacagtgaaccccatctctactaaaaatacaaaaattacccgggcatggtggcatgcacctgcagtgccagctactcgggaggctgaggcaggagaattgcttgaacccgggaggcggacgttgcagtgagcagagatcgcgccactgcactccagcctgggtgacagagcaggacaccgtctcagaaaaaaaaaaaaaagttacaactgaggcatcaggtcttaaggtttaaaacagtctcataattgtcacattatcatattatgtcaactctgaaaataaatgcacactcatcccagagtctccaaaatctttatctttagaatccaaccttgttttaagaagtagtaaaatgaaggagcattgttagtagtcacctgacaaaagctgtccattattcttgacattaaaaattgaatgcaatgatttaaaaaacataatacattaacatttacataatatatttagaatcacatggtttccagtgattagatttcagtcatgcctggaaaggagaagacagtggctaggagcacattccttataaaggatacataaatggtatacttaggatgactaatattaagaatttaaacacggtgcatttttttcctcaaaggaagcaattttagtttctaaagagcatttacttctgacatctcgattcctgatttcagtggctgcagactgtgtacttctgtgccacacttaggacaagtaaagtacacgtcaaataagaaactactcttagcacagaaataacagaaaatatgctcacatcctatggtgtgaggcatggtgggccactctccacatagagcgcattctttgccactggtggctaatgtattgtcactattaggtgcaccagtaagaggaatacaccatgaagacagcttggctttcaacttctggacattgataagtggtaagagaaaaatcagaaattcagcaaaaccatgccagagaagttccctattcatgtattcaaagccaacttcacatatgttttgaggcttgcaaaatacagaatgaatacctaggagacgttctgtcaaagttgcaaactttcccctctgaaggaaaatcaaaaaattaatcagcccacctaatttcaaaagtccaatcacaaaattcacacactgcttgactttcccaaatgatgctaaatgatggtttcgaaacaaatcatagcatcgttcttctaaccacctgccaccaattgtacaaacagcataccagattttttgatttttactgggtggctgatatctcaggttaggggaaaaatcatttttgtacttaatattcaaaactgactgtcccactgtggcatttttggagtagatggtgaatctccacaagaaaacccataagcacgctttcacctctggctcaaagcgagctaacagcccaggtttaaatccatgaaagcactgagtaaactgggaccaaactagctgctccagggccttgtttagttcaagtgcatccaactggcttattcttagcactctgtttgcactcttcgcattctcttttctggaagccatgtcttctctgaaggtctctttttcctgttcctgcagctccctcaagactggacagcctatagctatgacagtgggaatttttgctccaagttcttctgtgaaatccttgcctcatacttgccagaagcttaggagtctgcgaaacgcccacgctccacgtaactttctctgaaacattctctggaaagcttgtcttttcctagccgaatctggatt

SEQ ID NO: 16116 - RNA, 3541 nt, Homo sapiens
  source 1..3541: mol_type = other RNA
gctgggattacaggcatgagccattgtgtctagccatatctgcctttcagctagcctgctttgatctcccagttcccctgccctccctgctccctccccacaaggttcccatgcccatcaaacttggatagggagagaacaagcatatttaatttcttctagatctgcctgctttccttggtgcctgacccctgaccccgactgatttttccaacgcagtaaacatctctggcatcttatgggcgtgatccaggccagtgaggaatttggccaggaaagtcttttgtcatttgcaacctggttcgccctggaacagagggttggccaggagtgagatgccaagtggggggatttaaatggttctcctgaagtgacccctgaagccagatctgctgggacagatgtcctgggtgggcattgtgagtctggcctgttaggggcagttagcttcagatagcacctcaatttcaggtgagcctcaacttcccagtgggctctgctgcaaaaatgtggggtggggttccagggatggttttgtggtcctggaaatcactaaacagtatgcaaagtgggtaaacatgggcaatatgtgtggggtttttttggattccatgcttgcatcagaacccctgggggggaagtgctccagaaaactgtaaagtgcctgtccaggactggatgatcaggaccacagggacataaaggccaacatgattcttttccccaaacacttcttatcccaggatatcagctactagaccacagggatcaacctgcccaacttattcctgcaagcaagtatgtgcttaagttgtattttgttttgtttttaaacatgatacacctttatccagggaaggcagagaacagtcaagttattccagccacagaggaagggaataccagggtgtgagcctctcttgccaaaagccttagagaatctggaagaaattcttggctgtggagcagcaagaacgtgggccttggagctggacagccttggcccaggttcatgtccttgctctgccatgtacttcccaggacctctcagtgggtccctgggccagcagcctcgcgttccctgggagcttgttagagcacagagcccactgagtcagatgtgcttttttttttttttttttttgagatggagtttcactcttgtcccccaggctggagtgcagtggcacgatctctgctcactgcaacctctgcctcccaagttcaagcgattctggtgcctcagcctccgagtagctgggattacaggtgtgcaccaccgcgcctggcctaatttttgtatttttaatagagacggggtttccccatgttggccaggctggtctcgaactcctgacctcaggtgagccacccgccttggcctcccaaagtgctgggattacaagcgtgagccgccgcgcccggccagatgtacatttttaactggacctccaggtgactcttagcatgttcaggtttgaggagcactgacctgggaccctgggcaagtcgagtcaaataactccagcgtgcctcacggtcctcaacctgtcgcatggtgataatgcctacttgaaaaggtcgttgtgataattcaatgagataatgtattccagcacttagcacagtgcctggtacataggagatgttccatattcatctcctgatggtggaccttctttcgggaagtttaaatttcttttccactctcaaaaacgcctcttggttttgaacttgaagctgttgcagtgctggagtcggacagtagagggcactctcggcattgccatcgcggagagcaagacacgcgggatggaggctgcgtgggtccggacttcgtgtgtgcaggtgctgcgggccggctcctgggcacccacccagctcattcgccgagcggctcccctcctggggttgagtgtcctgggcctgagtctgcagcctcagccatctgttccccaacttgatctcccactgctagttacaaacaaatcgcccggcttgtgcaaacctcctgggctcagtccccagtcccgcggggccgctagacgttgatgaaggatccctggtcgccgttggccgtctcgggctccacacagcgccctttcctccgtgtaaccctgcggttccggtggaatttggcatagcagcgcagcccttccacacacatgcagtcatcgaagcatttgttgttgaggcctcggttgtggggtgtgcagagatgctcccgcaggtcgcagcaagtccctggcaggcagtcttggtgatggtcgcatggttccccttcggctggtgatgtttcgttaccatcactggagagtttaccgcggtgtttctctttcttctttgcagagggccaaccatcaggttttaagtcttcataatcggtccagtcgaacaaggccatgtccagcgtgggcatcacctccccgtcagacctgggctgtgcctgctggggccgcagggaggtgacgggcaggatcagggactcttctgtggcaggtgctgcctcaaaggtggtgagaaagaacatggtgggcgccaggctggtggaggattcctccatggctgcatccagcacctgggcttcggagagctctgccttcttcatcagggagctgggacctcggaccaaggctcggccttggtgcagcctcaacctgtccctgcgtctcttgtgctccctgctgcgtttcctggtcctctcccaacctggaggtcggttctccttctcggggtagggcaatgccagtcccaggagcaggtccttgtcctgcagcaggcctgcaggactctgctcaggcagcagcccctcagcctctggcagcctggaggcctgcctggtggcggtgaccacagccccatcctgggcctggctgggcaggcctgggccccactccttcttgcccgggccccgccggcggtggtggctggcctgaggcgtccacagcgctgggcctgggaggtcaatgtgattctcagggaggttccgggcaggggtcccaggtgcaagggcgcctgccaggctcagctccaggggcagcaggaggacgaggaacagcatgggagcggtgtggatggcaggcccagccattggctcctccctgggcctgggagagggggcagtgtgcagccagcatgatttgcgtcgccaaggatagagctgtgggccagtattcatgagccaggagaaaaaccttggagtctctggttcaaatgctgctactgtggctgtcccctggctgggtgatcttccgatgtgcttggagctggggtgacacaatatgaaaaggtggatgttaggagaggcctggactcctatcccatccagtttatgatgactttagggcctcagtttccttgtctgtaaaatgaggtacttgaggggccaaagcaggctccaatattcatcaactgatgactggataagcagatgtggtctatccatacacgggagtattttggttcttgtggcccaggatggcttctgaatatatctggacactcctgatgttgtgtaaggcatttagtgtctctgggccgg

SEQ ID NO: 16117 - RNA, 3405 nt, Homo sapiens
  source 1..3405: mol_type = other RNA
gctgggattacaggcatgagccattgtgtctagccatatctgcctttcagctagcctgctttgatctcccagttcccctgccctccctgctccctccccacaaggttcccatgcccatcaaacttggatagggagagaacaagcatatttaatttcttctagatctgcctgctttccttggtgcctgacccctgaccccgactgatttttccaacgcagtaaacatctctggcatcttatgggcgtgatccaggccagtgaggaatttggccaggaaagtcttttgtcatttgcaacctggttcgccctggaacagagggttggccaggagtgagatgccaagtggggggatttaaatggttctcctgaagtgacccctgaagccagatctgctgggacagatgtcctgggtgggcattgtgagtctggcctgttaggggcagttagcttcagatagcacctcaatttcaggtgagcctcaacttcccagtgggctctgctgcaaaaatgtggggtggggttccagggatggttttgtggtcctggaaatcactaaacagtatgcaaagtgggtaaacatgggcaatatgtgtggggtttttttggattccatgcttgcatcagaacccctgggggggaagtgctccagaaaactgtaaagtgcctgtccaggactggatgatcaggaccacagggacataaaggccaacatgattcttttccccaaacacttcttatcccaggatatcagctactagaccacagggatcaacctgcccaacttattcctgcaagcaagtatgtgcttaagttgtattttgttttgtttttaaacatgatacacctttatccagggaaggcagagaacagtcaagttattccagccacagaggaagggaataccagggtgtgagcctctcttgccaaaagccttagagaatctggaagaaattcttggctgtggagcagcaagaacgtgggccttggagctggacagccttggcccaggttcatgtccttgctctgccatgtacttcccaggacctctcagtgggtccctgggccagcagcctcgcgttccctgggagcttgttagagcacagagcccactgagtcagatgtgcttttttttttttttttttttgagatggagtttcactcttgtcccccaggctggagtgcagtggcacgatctctgctcactgcaacctctgcctcccaagttcaagcgattctggtgcctcagcctccgagtagctgggattacaggtgtgcaccaccgcgcctggcctaatttttgtatttttaatagagacggggtttccccatgttggccaggctggtctcgaactcctgacctcaggtgagccacccgccttggcctcccaaagtgctgggattacaagcgtgagccgccgcgcccggccagatgtacatttttaactggacctccaggtgactcttagcatgttcaggtttgaggagcactgacctgggaccctgggcaagtcgagtcaaataactccagcgtgcctcacggtcctcaacctgtcgcatggtgataatgcctacttgaaaaggtcgttgtgataattcaatgagataatgtattccagcacttagcacagtgcctggtacataggagatgttccatattcatctcctgatggtggaccttctttcgggaagtttaaatttcttttccactctcaaaaacgcctcttggttttgaacttgaagctgttgcagtgctggagtcggacagtagagggcactctcggcattgccatcgcggagagcaagacacgcgggatggaggctgcgtgggtccggacttcgtgtgtgcaggtgctgcgggccggctcctgggcacccacccagctcattcgccgagcggctcccctcctggggttgagtgtcctgggcctgagtctgcagcctcagccatctgttccccaacttgatctcccactgctagttacaaacaaatcgcccggcttgtgcaaacctcctgggctcagtccccagtcccgcggggccgctagacgttgatgaaggatccctggtcgccgttggccgtctcgggctccacacagcgccctttcctccgtgtaaccctgcggttccggtggaatttggcatagcagcgcagcccttccacacacatgcagtcatcgaagcatttgttgttgaggcctcggttgtggggtgtgcagagatgctcccgcaggtcgcagcaagtccctggcaggcagtcttggtgatggtcgcatggttccccttcggctggtgatgtttcgttaccatcactggagagtttaccgcggtgtttctctttcttctttgcagagggccaaccatcaggttttaagtcttcataatcggtccagtcgaacaaggccatgtccagcgtgggcatcacctccccgtcagacctgggctgtgcctgctggggccgcagggaggtgacgggcaggatcagggactcttctgtggcaggtgctgcctcaaaggtggtgagaaagaacatggtgggcgccaggctggtggaggattcctccatggctgcatccagcacctgggcttcggagagctctgccttcttcatcagggagctgggacctcggaccaaggctcggccttggtgcagcctcaacctgtccctgcgtctcttgtgctccctgctgcgtttcctggtcctctcccaacctggaggtcggttctccttctcggggtagggcaatgccagtcccaggagcaggtccttgtcctgcagcaggcctgcaggactctgctcaggcagcagcccctcagcctctggcagcctggaggcctgcctggtggcggtgaccacagccccatcctgggcctggctgggcaggcctgggccccactccttcttgcccgggccccgccggcggtggtggctggcctgaggcgtccacagcgctgggcctgggaggtcaatgtgattctcagggaggttccgggcaggggtcccaggtgcaagggcgcctgccaggctcagctccaggggcagcaggaggacgaggaacagcatgggagcggtgtggatggcaggcccagccattggctcctccctgggcctgggagagggggcagtgtgcagccagcatgatttgcgtcgccaaggatagagctgtgggccagtattcatgagccaggagaaaaaccttggagtctctggttcaaatgctgctactgtggctgtcccctggctgggtgatcttccgatgtgcttggagcttgtggcccaggatggcttctgaatatatctggacactcctgatgttgtgtaaggcatttagtgtctctgggccgggcgcagtggctcaagcctgtaatcccaacactttggcaggtggaggcgggcacatcacttgg

SEQ ID NO: 16118 - RNA, 3245 nt, Homo sapiens
  source 1..3245: mol_type = other RNA
gctgggattacaggcatgagccattgtgtctagccatatctgcctttcagctagcctgctttgatctcccagttcccctgccctccctgctccctccccacaaggttcccatgcccatcaaacttggatagggagagaacaagcatatttaatttcttctagatctgcctgctttccttggtgcctgacccctgaccccgactgatttttccaacgcagtaaacatctctggcatcttatgggcgtgatccaggccagtgaggaatttggccaggaaagtcttttgtcatttgcaacctggttcgccctggaacagagggttggccaggagtgagatgccaagtggggggatttaaatggttctcctgaagtgacccctgaagccagatctgctgggacagatgtcctgggtgggcattgtgagtctggcctgttaggggcagttagcttcagatagcacctcaatttcaggtgagcctcaacttcccagtgggctctgctgcaaaaatgtggggtggggttccagggatggttttgtggtcctggaaatcactaaacagtatgcaaagtgggtaaacatgggcaatatgtgtggggtttttttggattccatgcttgcatcagaacccctgggggggaagtgctccagaaaactgtaaagtgcctgtccaggactggatgatcaggaccacagggacataaaggccaacatgattcttttccccaaacacttcttatcccaggatatcagctactagaccacagggatcaacctgcccaacttattcctgcaagcaagtatgtgcttaagttgtattttgttttgtttttaaacatgatacacctttatccagggaaggcagagaacagtcaagttattccagccacagaggaagggaataccagggtgtgagcctctcttgccaaaagccttagagaatctggaagaaattcttggctgtggagcagcaagaacgtgggccttggagctggacagccttggcccaggttcatgtccttgctctgccatgtacttcccaggacctctcagtgggtccctgggccagcagcctcgcgttccctgggagcttgttagagcacagagcccactgagtcagatgtgcttttttttttttttttttttgagatggagtttcactcttgtcccccaggctggagtgcagtggcacgatctctgctcactgcaacctctgcctcccaagttcaagcgattctggtgcctcagcctccgagtagctgggattacaggtgtgcaccaccgcgcctggcctaatttttgtatttttaatagagacggggtttccccatgttggccaggctggtctcgaactcctgacctcaggtgagccacccgccttggcctcccaaagtgctgggattacaagcgtgagccgccgcgcccggccagatgtacatttttaactggacctccaggtgactcttagcatgttcaggtttgaggagcactgacctgggaccctgggcaagtcgagtcaaataactccagcgtgcctcacggtcctcaacctgtcgcatggtgataatgcctacttgaaaaggtcgttgtgataattcaatgagataatgtattccagcacttagcacagtgcctggtacataggagatgttccatattcatctcctgatggtggaccttctttcgggaagtttaaatttcttttccactctcaaaaacgcctcttggttttgaacttgaagctgttgcagtgctggagtcggacagtagagggcactctcggcattgccatcgcggagagcaagacacgcgggatggaggctgcgtgggtccggacttcgtgtgtgcaggtgctgcgggccggctcctgggcacccacccagctcattcgccgagcggctcccctcctggggttgagtgtcctgggcctgagtctgcagcctcagccatctgttccccaacttgatctcccactgctagttacaaacaaatcgcccggcttgtgcaaacctcctgggctcagtccccagtcccgcggggccgctagacgttgatgaaggatccctggtcgccgttggccgtctcgggctccacacagcgccctttcctccgtgtaaccctgcggttccggtggaatttggcatagcagcgcagcccttccacacacatgcagtcatcgaagcatttgttgttgaggcctcggttgtggggtgtgcagagatgctcccgcaggtcgcagcaagtccctggcaggcagtcttggtgatggtcgcatggttccccttcggctggtgatgtttcgttaccatcactggagagtttaccgcggtgtttctctttcttctttgcagagggccaaccatcaggttttaagtcttcataatcggtccagtcgaacaaggccatgtccagcgtgggcatcacctccccgtcagacctgggctgtgcctgctggggccgcagggaggtgacgggcaggatcagggactcttctgtggcaggtgctgcctcaaaggtggtgagaaagaacatggtgggcgccaggctggtggaggattcctccatggctgcatccagcacctgggcttcggagagctctgccttcttcatcagggagctgggacctcggaccaaggctcggccttggtgcagcctcaacctgtccctgcgtctcttgtgctccctgctgcgtttcctggtcctctcccaacctggaggtcggttctccttctcggggtagggcaatgccagtcccaggagcaggtccttgtcctgcagcaggcctgcaggactctgctcaggcagcagcccctcagcctctggcagcctggaggcctgcctggtggcggtgaccacagccccatcctgggcctggctgggcaggcctgggccccactccttcttgcccgggccccgccggcggtggtggctggcctgaggcgtccacagcgctgggcctgggaggtcaatgtgattctcagggaggttccgggcaggggtcccaggtgcaagggcgcctgccaggctcagctccaggggcagcaggaggacgaggaacagcatgggagcggtgtggatggcaggcccagccattggctcctccctgtccggccggcgggtagggggaggaggggctcggggccgagcgcccgcgggagccgagcgcagccgagggcgagccgcggaacggggccggcgtggagaggtgcgcgggcagccggaggatgtgcccgggctgagcgggact

SEQ ID NO: 16119 - RNA, 2856 nt, Homo sapiens
  source 1..2856: mol_type = other RNA
gctgggattacaggcatgagcccaccgcgcctggctatttcttttctgaaagataattttaagaccctattcaatccagactctttttatcatagagcaagatttgattttcaattttttccttcaacctttccaattccttaaaactacagactttcttgcttttaatccttagcttactagttcttggcctatgcagaaatgcaacttctcctcttacacagtatacttattcaatattattactgctattggtcatgcttttcttagttaataatgctaatacgtactgtctttcccagtggtatttctattttaaactctgctataactatggagtaaaactttgggctctcaagaggatttcaaatctcagctgtctgcctggggactttaaaatataaccattttttaaaaacttataaaaatttccaacacaaagtagaatatagtcattacacagattcaacattaacaggatttttgtcacatttccttaatcgattccttgtttctctgctgaatacttcagagcaaatctatcatgtcatttaaaaactctatgtagcacaatatacctctcttaaaagggagggaccatgttcttatataatcaaaatgcaagtagcttatataatctaatagaattaacaataactcttttgtttggggacctctgaagtgaaacaaatcatacagaattttaatactataaaaacattagcactgtaaaaacagcaacatattatacagcctcaaaacagttttaaactgaagtctagtatgttcagaaacgcagggtgctgacccaccatccaactgaagctgagctcaggaatgcctaagacaactcataaaaatacacagcatcaagatcagtctttgtacattatttcaatgaaaaacacatagctgtgtacaaatatacagatctcaaactgtaacactgaaacacaaaatgcaacaaagtggctttataagttttcttcactgagacagaccttctggtgacttctggtgaatctagacatttatgattattaatacataataagcaagagaaatacagattttccaacctcatgatcagtaaattcctttgaaaaatgaatgaaggtatcagagtcatcaaaaggggaaacagttggtaagtttgatggccctgcctacactgtataatgtaagacacacaataagagctataagaaactatagttaaatgttagaagtaaagccaatatcgttttctcagacttctcccagtgattatatacctgatatataaacatcttcaaatgtgaaatagttcaataacacaatgacactttgccagtgtattaatctgatatatattttgaactggaatgatttgtaaagaaataaataagaaaccctaaaaagaaaccattagttccaagtcaaattatgttaatggtctatagaaaaaagtgagtgtgggcaggaaacattggctacatgccaatttttatttcaaagagtaatgttgcacaaataatagttatcattgtcttacacaacaaaaaatcctaaagttaatctcacaaacctaaattagctgaacatggagtaacaaagtcaaagccagtattatcatcagcacattaatttgataaatcaaactacatctttaaaaaaaaaccctgcatctgctgctgtgcagaactgataattacttttcagcatgtaaacgaaaaatcattatacagctctctctcttttttttttttttcctagaaagatgtataccagggaaacacaacagaatttgttacttgttaaatcccacaaaagctacaagggagctgagagttgatggcacttaaggacagtaaaagtctgcacttttaatatttttaatgcccactgatgggctttgtgtcaatactttttaaaatgctttttatttacaatagataaaacagtaaggaaatacaatattatatcatatccccgcacagagatactatatctgtataaatgaatcactagtaaaagagttatttcttatttcaaatgaagtcttatctaggtattaattaggctgtaatctaaatgttgatggtgcctattttcaactcccaaaataaacagaaagagctcatgtatcaagattaattttctttggccgcaatggataccattttctctgggggcagtctttagtttgctttcttttcagtaccatgtcagaggttttcctggaagcagtctctgttggtgtggtttctatctgtgttataaagttctcaggtttagcatctggtttcctatgacaactggaaaagacttcttggtgaatcctctggaggtggataacaggctgcatcctgagaacttgggaaaatccctctccttgttcaattaatgcaggcaaggacagaatttcttgttttgcttttatggttttgatgacacattccaggatctttctgggatactgcttacgttttgtggctatatctactatgatttcatcaaactgatcttcaagtactttgatgtcagaatccataaaacaattatctgaagcttcctgccatgcttgcccattaatgctgatattctcttgcacagctgattcaaaagtccactgcgcatctcgcagagcgggctcccgaatctcctccggcagagcgtccccgagcttttgcacgaagcggccgcacagttgtagcatttcggtcacagcccgcttcgaggtgcagcgcacccgaaagtcttctcggggagtggcggagaccaaggcctggctctctgtgccagccgcgagctccttgtcccatggagggtcaaggaccaccaactcaggagaccccgccatttttcgtcggaact

SEQ ID NO: 16120 - RNA, 2911 nt, Homo sapiens
  source 1..2911: mol_type = other RNA
gctgggattacaggcatgagcccaccgcgcctggctatttcttttctgaaagataattttaagaccctattcaatccagactctttttatcatagagcaagatttgattttcaattttttccttcaacctttccaattccttaaaactacagactttcttgcttttaatccttagcttactagttcttggcctatgcagaaatgcaacttctcctcttacacagtatacttattcaatattattactgctattggtcatgcttttcttagttaataatgctaatacgtactgtctttcccagtggtatttctattttaaactctgctataactatggagtaaaactttgggctctcaagaggatttcaaatctcagctgtctgcctggggactttaaaatataaccattttttaaaaacttataaaaatttccaacacaaagtagaatatagtcattacacagattcaacattaacaggatttttgtcacatttccttaatcgattccttgtttctctgctgaatacttcagagcaaatctatcatgtcatttaaaaactctatgtagcacaatatacctctcttaaaagggagggaccatgttcttatataatcaaaatgcaagtagcttatataatctaatagaattaacaataactcttttgtttggggacctctgaagtgaaacaaatcatacagaattttaatactataaaaacattagcactgtaaaaacagcaacatattatacagcctcaaaacagttttaaactgaagtctagtatgttcagaaacgcagggtgctgacccaccatccaactgaagctgagctcaggaatgcctaagacaactcataaaaatacacagcatcaagatcagtctttgtacattatttcaatgaaaaacacatagctgtgtacaaatatacagatctcaaactgtaacactgaaacacaaaatgcaacaaagtggctttataagttttcttcactgagacagaccttctggtgacttctggtgaatctagacatttatgattattaatacataataagcaagagaaatacagattttccaacctcatgatcagtaaattcctttgaaaaatgaatgaaggtatcagagtcatcaaaaggggaaacagttggtaagtttgatggccctgcctacactgtataatgtaagacacacaataagagctataagaaactatagttaaatgttagaagtaaagccaatatcgttttctcagacttctcccagtgattatatacctgatatataaacatcttcaaatgtgaaatagttcaataacacaatgacactttgccagtgtattaatctgatatatattttgaactggaatgatttgtaaagaaataaataagaaaccctaaaaagaaaccattagttccaagtcaaattatgttaatggtctatagaaaaaagtgagtgtgggcaggaaacattggctacatgccaatttttatttcaaagagtaatgttgcacaaataatagttatcattgtcttacacaacaaaaaatcctaaagttaatctcacaaacctaaattagctgaacatggagtaacaaagtcaaagccagtattatcatcagcacattaatttgataaatcaaactacatctttaaaaaaaaaccctgcatctgctgctgtgcagaactgataattacttttcagcatgtaaacgaaaaatcattatacagctctctctcttttttttttttttcctagaaagatgtataccagggaaacacaacagaatttgttacttgttaaatcccacaaaagctacaagggagctgagagttgatggcacttaaggacagtaaaagtctgcacttttaatatttttaatgcccactgatgggctttgtgtcaatactttttaaaatgctttttatttacaatagataaaacagtaaggaaatacaatattatatcatatccccgcacagagatactatatctgtataaatgaatcactagtaaaagagttatttcttatttcaaatgaagtcttatctaggtattaattaggctgtaatctaaatgttgatggtgcctattttcaactcccaaaataaacagaaagagctcatgtatcaagattaattttctttggccgcaatggataccattttctctgggggcagtctttagtttgctttcttttcagtaccatgtcagaggttttcctggaagcagtctctgttggtgtggtttctatctgtgttataaagttctcaggtttagcatctggtttcctatgacaactggaaaagacttcttggtgaatcctctggaggtggataacaggctgcatcctgagaacttgggaaaatccctctccttgttcaattaatgcaggcaaggactggatcagggtcatattttaggtccagtggatgtacaacagggtggtactgcttcagaatttcttgttttgcttttatggttttgatgacacattccaggatctttctgggatactgcttacgttttgtggctatatctactatgatttcatcaaactgatcttcaagtactttgatgtcagaatccataaaacaattatctgaagcttcctgccatgcttgcccattaatgctgatattctcttgcacagctgattcaaaagtccactgcgcatctcgcagagcgggctcccgaatctcctccggcagagcgtccccgagcttttgcacgaagcggccgcacagttgtagcatttcggtcacagcccgcttcgaggtgcagcgcacccgaaagtcttctcggggagtggcggagaccaaggcctggctctctgtgccagccgcgagctccttgtcccatggagggtcaaggaccaccaactcaggagaccccgccatttttcgtcggaact

SEQ ID NO: 16121 - RNA, 3064 nt, Homo sapiens
  source 1..3064: mol_type = other RNA
gctgggattacaggcatgagcccaccgcgcctggctatttcttttctgaaagataattttaagaccctattcaatccagactctttttatcatagagcaagatttgattttcaattttttccttcaacctttccaattccttaaaactacagactttcttgcttttaatccttagcttactagttcttggcctatgcagaaatgcaacttctcctcttacacagtatacttattcaatattattactgctattggtcatgcttttcttagttaataatgctaatacgtactgtctttcccagtggtatttctattttaaactctgctataactatggagtaaaactttgggctctcaagaggatttcaaatctcagctgtctgcctggggactttaaaatataaccattttttaaaaacttataaaaatttccaacacaaagtagaatatagtcattacacagattcaacattaacaggatttttgtcacatttccttaatcgattccttgtttctctgctgaatacttcagagcaaatctatcatgtcatttaaaaactctatgtagcacaatatacctctcttaaaagggagggaccatgttcttatataatcaaaatgcaagtagcttatataatctaatagaattaacaataactcttttgtttggggacctctgaagtgaaacaaatcatacagaattttaatactataaaaacattagcactgtaaaaacagcaacatattatacagcctcaaaacagttttaaactgaagtctagtatgttcagaaacgcagggtgctgacccaccatccaactgaagctgagctcaggaatgcctaagacaactcataaaaatacacagcatcaagatcagtctttgtacattatttcaatgaaaaacacatagctgtgtacaaatatacagatctcaaactgtaacactgaaacacaaaatgcaacaaagtggctttataagttttcttcactgagacagaccttctggtgacttctggtgaatctagacatttatgattattaatacataataagcaagagaaatacagattttccaacctcatgatcagtaaattcctttgaaaaatgaatgaaggtatcagagtcatcaaaaggggaaacagttggtaagtttgatggccctgcctacactgtataatgtaagacacacaataagagctataagaaactatagttaaatgttagaagtaaagccaatatcgttttctcagacttctcccagtgattatatacctgatatataaacatcttcaaatgtgaaatagttcaataacacaatgacactttgccagtgtattaatctgatatatattttgaactggaatgatttgtaaagaaataaataagaaaccctaaaaagaaaccattagttccaagtcaaattatgttaatggtctatagaaaaaagtgagtgtgggcaggaaacattggctacatgccaatttttatttcaaagagtaatgttgcacaaataatagttatcattgtcttacacaacaaaaaatcctaaagttaatctcacaaacctaaattagctgaacatggagtaacaaagtcaaagccagtattatcatcagcacattaatttgataaatcaaactacatctttaaaaaaaaaccctgcatctgctgctgtgcagaactgataattacttttcagcatgtaaacgaaaaatcattatacagctctctctcttttttttttttttcctagaaagatgtataccagggaaacacaacagaatttgttacttgttaaatcccacaaaagctacaagggagctgagagttgatggcacttaaggacagtaaaagtctgcacttttaatatttttaatgcccactgatgggctttgtgtcaatactttttaaaatgctttttatttacaatagataaaacagtaaggaaatacaatattatatcatatccccgcacagagatactatatctgtataaatgaatcactagtaaaagagttatttcttatttcaaatgaagtcttatctaggtattaattaggctgtaatctaaatgttgatggtgcctattttcaactcccaaaataaacagaaagagctcatgtatcaagattaattttctttggccgcaatggataccattttctctgggggcagtctttagtttgctttcttttcagtaccatgtcagaggttttcctggaagcagtctctgttggtgtggtttctatctgtgttataaagttctcaggtttagcatctggtttcctatgacaactggaaaagacttcttggtgaatcctctggaggtggataacaggctgcatcctgagaacttgggaaaatccctctccttgttcaattaatgcaggcaaggacttcatggcttcactgatctcctttgctactgtttcccctctgcatttcaaattttccatatgaggggctcgaagtaataaaaaccatatatgacaaatccacagccaacatcatgttgaatggggaaaagttgaaagcattcccgttgagaactggatcagggtcatattttaggtccagtggatgtacaacagggtggtactgcttcagaatttcttgttttgcttttatggttttgatgacacattccaggatctttctgggatactgcttacgttttgtggctatatctactatgatttcatcaaactgatcttcaagtactttgatgtcagaatccataaaacaattatctgaagcttcctgccatgcttgcccattaatgctgatattctcttgcacagctgattcaaaagtccactgcgcatctcgcagagcgggctcccgaatctcctccggcagagcgtccccgagcttttgcacgaagcggccgcacagttgtagcatttcggtcacagcccgcttcgaggtgcagcgcacccgaaagtcttctcggggagtggcggagaccaaggcctggctctctgtgccagccgcgagctccttgtcccatggagggtcaaggaccaccaactcaggagaccccgccatttttcgtcggaact

SEQ ID NO: 16122 - RNA, 2979 nt, Homo sapiens
  source 1..2979: mol_type = other RNA
gctgggattacaggcatgagcccaccgcgcctggctatttcttttctgaaagataattttaagaccctattcaatccagactctttttatcatagagcaagatttgattttcaattttttccttcaacctttccaattccttaaaactacagactttcttgcttttaatccttagcttactagttcttggcctatgcagaaatgcaacttctcctcttacacagtatacttattcaatattattactgctattggtcatgcttttcttagttaataatgctaatacgtactgtctttcccagtggtatttctattttaaactctgctataactatggagtaaaactttgggctctcaagaggatttcaaatctcagctgtctgcctggggactttaaaatataaccattttttaaaaacttataaaaatttccaacacaaagtagaatatagtcattacacagattcaacattaacaggatttttgtcacatttccttaatcgattccttgtttctctgctgaatacttcagagcaaatctatcatgtcatttaaaaactctatgtagcacaatatacctctcttaaaagggagggaccatgttcttatataatcaaaatgcaagtagcttatataatctaatagaattaacaataactcttttgtttggggacctctgaagtgaaacaaatcatacagaattttaatactataaaaacattagcactgtaaaaacagcaacatattatacagcctcaaaacagttttaaactgaagtctagtatgttcagaaacgcagggtgctgacccaccatccaactgaagctgagctcaggaatgcctaagacaactcataaaaatacacagcatcaagatcagtctttgtacattatttcaatgaaaaacacatagctgtgtacaaatatacagatctcaaactgtaacactgaaacacaaaatgcaacaaagtggctttataagttttcttcactgagacagaccttctggtgacttctggtgaatctagacatttatgattattaatacataataagcaagagaaatacagattttccaacctcatgatcagtaaattcctttgaaaaatgaatgaaggtatcagagtcatcaaaaggggaaacagttggtaagtttgatggccctgcctacactgtataatgtaagacacacaataagagctataagaaactatagttaaatgttagaagtaaagccaatatcgttttctcagacttctcccagtgattatatacctgatatataaacatcttcaaatgtgaaatagttcaataacacaatgacactttgccagtgtattaatctgatatatattttgaactggaatgatttgtaaagaaataaataagaaaccctaaaaagaaaccattagttccaagtcaaattatgttaatggtctatagaaaaaagtgagtgtgggcaggaaacattggctacatgccaatttttatttcaaagagtaatgttgcacaaataatagttatcattgtcttacacaacaaaaaatcctaaagttaatctcacaaacctaaattagctgaacatggagtaacaaagtcaaagccagtattatcatcagcacattaatttgataaatcaaactacatctttaaaaaaaaaccctgcatctgctgctgtgcagaactgataattacttttcagcatgtaaacgaaaaatcattatacagctctctctcttttttttttttttcctagaaagatgtataccagggaaacacaacagaatttgttacttgttaaatcccacaaaagctacaagggagctgagagttgatggcacttaaggacagtaaaagtctgcacttttaatatttttaatgcccactgatgggctttgtgtcaatactttttaaaatgctttttatttacaatagataaaacagtaaggaaatacaatattatatcatatccccgcacagagatactatatctgtataaatgaatcactagtaaaagagttatttcttatttcaaatgaagtcttatctaggtattaattaggctgtaatctaaatgttgatggtgcctattttcaactcccaaaataaacagaaagagctcatgtatcaagattaattttctttggccgcaatggataccattttctctgggggcagtctttagtttgctttcttttcagtaccatgtcagaggttttcctggaagcagtctctgttggtgtggtttctatctgtgttataaagttctcaggtttagcatctggtttcctatgacaactggaaaagacttcttggtgaatcctctggaggtggataacaggctgcatcctgagaacttgggaaaatccctctccttgttcaattaatgcaggcaaggacttcatggcttcactgatctcctttgctactgtttcccctctgcatttcaaattttccatatgaggggctggatcagggtcatattttaggtccagtggatgtacaacagggtggtactgcttcagaatttcttgttttgcttttatggttttgatgacacattccaggatctttctgggatactgcttacgttttgtggctatatctactatgatttcatcaaactgatcttcaagtactttgatgtcagaatccataaaacaattatctgaagcttcctgccatgcttgcccattaatgctgatattctcttgcacagctgattcaaaagtccactgcgcatctcgcagagcgggctcccgaatctcctccggcagagcgtccccgagcttttgcacgaagcggccgcacagttgtagcatttcggtcacagcccgcttcgaggtgcagcgcacccgaaagtcttctcggggagtggcggagaccaaggcctggctctctgtgccagccgcgagctccttgtcccatggagggtcaaggaccaccaactcaggagaccccgccatttttcgtcggaact

SEQ ID NO: 16123 - RNA, 1803 nt, Homo sapiens
  source 1..1803: mol_type = other RNA
gctgggattacaggcatgagccccacgcacggccaaatctctggttatcttttctaacctctaaattcacattcccttggtttagtgtttactgctcttatgaagtgagagaaaccccacttggcaaaagcacgttggtatttcctagagaggctctgggttttgcttttgtttttgtttttgtttttttaagttgttgtttgtttgtttttactttcatctgttttaaagtttccatggtagcatggtagattgtggtctattgagcagtcagaaagcctgggtttgatttctggtctgcactaacctgctatgtgctcctgtgcattccgatttacctcactgaggccgtttcttcatgaggagaaactcaatgaggaaatttgtgttaaatcagattatcaagagttgcagtattatataaagccaacggaagcaaggctgttttggttggatttgaagaggaaccatggacgcacatcctttcttgcccatctgcatggcctgagaataaccttcatatcctctccaaggaactctaggattcctatgtagaaagtagccagaaaatgatcagtcctgatggtttcgaagatctcaaactgtaccattcaatagttctatacctggcagaaggtcagtgcatctctcccttgcagccagtcccgggaaacaggtctctgaaagaatggaagcctttcaaattctttttttatggagatggctggcagccaaaggagcaggattatagagaccccaaactagactgaagggattgagggacaaatgagaaaggggaatgtcaaggcaaattttcacaatggcttgcactattccaagtaacaggaactaatttatctcagaaacaccgggcttactgctaaaaccaacactgctttctagctcgttcctaataacacccatttctgggctttctaacatcctatttggtcattaatagcagccttcacagaaacataaatgaaactaagaattgaatatttatatttatgatgtaaaataaaattactttcccaagtgtttcagccaagtgttgacaggaaataaaacagaattcacagggatagtggattttctgacaagtttgagatgtcagcatcgcacgctttcaggcaaagtgcaacagaaggaactgtacttgtcattacaccaactgcctccttcccagtggagggtctttgatcctggtactatgactcactgggtcactaaggacttcagttgtccctccaccatggtgggtcttgggtttctccattcagtccagataacacatgtaaaggatctgaggtccctagataagaagcaacattcagtagaatttggcattcataggatgatgaaatttatgacatcattatcccagttctcacggttataatccacagaaagcttctctttattctcagaactagcccttgtagtggccttgaatgtgcaaacgttaccctttagtaatgtttgaggcagaatttgaaaatctgaaacatgattcaaagctaccctacaataactaagctgccatagttacctaaggctgcttcccaatatgttttctatgaatctgcctttccaatagagcacagtgcagggaaaaggggagggggcaattgtacaaaagacacaaaaggtccagttttagtttggcccatgactgccatgccctggaattctgtacagtctcagaaagagagtgtcactgattattaaaaatacataatttcttcttttttatttttttaatttttagaaacatgggtcttactatgttgcccaggatag

SEQ ID NO: 16124 - RNA, 3601 nt, Homo sapiens
  source 1..3601: mol_type = other RNA
gctgggattacaggcatgagccccacgcacggccaaatctctggttatcttttctaacctctaaattcacattcccttggtttagtgtttactgctcttatgaagtgagagaaaccccacttggcaaaagcacgttggtatttcctagagaggctctgggttttgcttttgtttttgtttttgtttttttaagttgttgtttgtttgtttttactttcatctgttttaaagtttccatggtagcatggtagattgtggtctattgagcagtcagaaagcctgggtttgatttctggtctgcactaacctgctatgtgctcctgtgcattccgatttacctcactgaggccgtttcttcatgaggagaaactcaatgaggaaatttgtgttaaatcagattatcaagagttgcagtattatataaagccaacggaagcaaggctgttttggttggatttgaagaggaaccatggacgcacatcctttcttgcccatctgcatggcctgagaataaccttcatatcctctccaaggaactctaggattcctatgtagaaagtagccagaaaatgatcagtcctgatggtttcgaagatctcaaactgtaccattcaatagttctatacctggcagaaggtcagtgcatctctcccttgctgatggttattcattcaaacatgaaaggagaaaataactggtttagtctttctcaggaacacacactctttttttagagtcagactattttcttcttcaatgagttaagttttactagagacacttagtagtatatttggaaacttaaaatgtaatagtagtacctcttcttttctgatcttctgtttattcccttacctacctaaaaagatcaatcacttactaggattaacccaacacttaggctcaatcaactgcatgaacgtgtttggactctcaaaatactatatttcctcaattttacaacatactttttttaaacatttaaaaatttctaatataatcattagtttaaatttttacgtaaaaagcctcaaatgccagggagtgaagagaggtggttctcattgcctgtgcatttgcaagcttagaaatgtctaaaggaaaggtatcttttcattcttcctcccaatcctttcattcatctaacaaactgttgttcactgagtgcctgttttgtatcacgtacatttctgggcacagggagtacagagtacaatgataggcaagcatcaatgatagactctcaaagagtctcattctagtagggaaaggtagatgataaacaattgaactgataaataaagaattttcaattgtgataaatgttacaaagaaagcaagacagaaagatcaggaagtggggtaagtcagggaggtttctctgattaaataacatgtaagcagaaagctgagtgctgagcagttgcaagggcagtccctgtagagaaaacagtaagtgcaggggccctggggcaagctggcctgagctcagcagaataagggaacatggagacaccctgttgactcatttacatggctagctgaacaagaagttccatttaacttaaatttggatttctatctcttaaacaaaatatctttcaaaagatacattatgatgctagactaaagctaacagagaaaaacgcagaactaaagtccattgtttctggtaaagcaatggcccgtttggtccccatatagagataaagctgtttaaatgcatcatggaaaaataggcccactctcatgatgaaaggcttatagggagccaaattcctttccaaagctgttattaaacagagcatctttttttttttctttttaatggttgcagcacaccaacatggcacaggtatacatatgtaacaaacctgcacgttgtgcacatttaccctagaacttaaagtatgataaaaaaaaaaaatgaaaagagcatcttaaaggactatctctatttccagcagaccttcaagagaagtttaaaggaatatgtaatgttatagtcaattctaaattactaaaaaggccagaagaggcagattactgcaaacagcctatctgagcactgcagtacacaattgtcaaggatcaaaatcagctcagaggaatcataaaactccaagaagccttcgaatcaaacatgaatggtgacagtgaagaagaaagagaaatgtcatcacatcaataaacataggctaagtgagtaaaggaagaaacgtgtgtacatttcctacaataaggttgttcccctcccaatcttgttattaaatccatagtgtgtcttacaaacatggactctcagaatcatagaaataccacagctctttctccagcctgctaaagtgcttggaatttccaccattaagctctaggaagttctgtaagaacattttatcaagaaatataacacagtaacacatcacaatctgtttgaaaaatgagcatgatttatcttaccagccagtcccgggaaacaggtctctgaaagaatggaagcctttcaaattctttttttatggagatggctggcagccaaaggagcaggattatagagaccccaaactagactgaagggattgagggacaaatgagaaaggggaatgtcaaggcaaattttcacaatggcttgcactattccaagtaacaggaactaatttatctcagaaacaccgggcttactgctaaaaccaacactgctttctagctcgttcctaataacacccatttctgggctttctaacatcctatttggtcattaatagcagccttcacagaaacataaatgaaactaagaattgaatatttatatttatgatgtaaaataaaattactttcccaagtgtttcagccaagtgttgacaggaaataaaacagaattcacagggatagtggattttctgacaagtttgagatgtcagcatcgcacgctttcaggcaaagtgcaacagaaggaactgtacttgtcattacaccaactgcctccttcccagtggagggtctttgatcctggtactatgactcactgggtcactaaggacttcagttgtccctccaccatggtgggtcttgggtttctccattcagtccagataacacatgtaaaggatctgaggtccctagataagaagcaacattcagtagaatttggcattcataggatgatgaaatttatgacatcattatcccagttctcacggttataatccacagaaagcttctctttattctcagaactagcccttgtagtggccttgaatgtgcaaacgttaccctttagtaatgtttgaggcagaatttgaaaatctgaaacatgattcaaagctaccctacaataactaagctgccatagttacctaaggctgcttcccaatatgttttctatgaatctgcctttccaatagagcacagtgcagggaaaaggggagggggcaattgtacaaaagacacaaaaggtccagttttagtttggcccatgactgccatgccctggaattctgtacagtctcagaaagagagtgtcactgattattaaaaatacataatttcttcttttttatttttttaatttttagaaacatgggtcttactatgttgccca

SEQ ID NO: 16125 - RNA, 7655 nt, Homo sapiens
  source 1..7655: mol_type = other RNA
gctgggattacaggcatgagcccccaagcctggccagaaagtatttccaagaactgagtgaatgtttatttctgaaaatgaatgatgaaaacgtgttcttccccttcacctcaataggtcttgacagggtctacagggggaatcccagagtgtgcccggcgctgacagcagcaagagacaggagctgggcagagcatccctggctaggggatctgccagagcctagctgacagcatcctctcttccctgccccctgaattcatcttcccctcctggccctgggcttccccatctctcttgctcctgcctgctgtgacagctaattgcaggatgcaattttctgcctcccatctccctatctgcatgtctccctacttcctttcagggtcatttttttttttttttaccttttttcttttttgagacagagtcttgctctgtcacccaggctagagtgcagtggtgtgatcttggctcactgcaacctctgcctcctgggcccaagagattctcctgcttcagcctctcaagtagctgggattacaggtgtgcaccaccgcacctgtctaatttctgtatttttagtagagacggggtttcaccatattggccaggctggtctcgaactcctgacctcaagtgatccacccacttcggcctcccaaagtgctgggattacacacgtgagccatcgcacctggcctttgtgtcagttacacacacacacacacacacacacacacacacacttgcctgaattccctttccttctgtcttccccccaaattctctctcccctccactccagcagggcttctgtccccaccactgcactgaactgacatcttatcttatcaagatcaccaaccctgtccatgtcatcagacctaatggtcactctgctctctgcatccttgtccaagtctcagcagcccttggcacagctggctgtctcctctccttcttgaaacacaaaggtgcatttgccctctgtaaccctcctggtttcagcctacctcgagatcactcctaagctcgttttgctacatccccttctcccccagatgtagatgtccccaaggctctggccagggtcgcttctctgtccccacccccctgctaggccacgtcacccaatcctgtggctttatgttgacgtttccaaaacttacgtttttgagccacggcctctctttcccccaaactccagtctcacatatccaactggctatttgataccacaactcggatttctcgaaggcagatctatcttgacacatccaaaagagaagccttggttcctccctcccaaagccactttcctgatcccagtctcctcgttcctggtaacaatcctcatcggtgcccatcagagatgtgcgtgcccaattcagagagttcttctcttcctggttccttttccttccctcctctatgacatccagttcaccaccaatgcaggctctagcctccaaaatcccatgccttcttccacttcctccatcccactaactccaccttggtccaggcctccagcaaccagaggaaggcaacagcccgctacctccttccttcccctttgactcctgaagtctacgtatgctcagcacagcaatgtaattctgctgttcttgtttaaataaaaatatgaggccgggcgcagtggctcactcctgtaatcccagcattttgggaggccgaggcaggtggatcatttgaagccaggaatttcagattggcctggccaacacggtgaaatcccgtctttactaaaaatacaaaaaaattagccaggcgtggtggcacatgcctgtaatcccagctactcaggaggctgaggcaggagaatcacttgaacttgggaggcggaggttggcagtgagccgagatcagcccactggactccagcctgagacagagcaagactctttttcaaaataaatataaataagaaaataaaaatatgatcatggcatgcctgtgctcaaaaccctccaagcacttcccatcagatctagaataaaattcagatttcttcccaaggatccaaggccctaactgatcagcccctaccctgtgcctctgtcctatggtggatctgctcaccgcacaggcctcctcgaagacctgctacttttctgggctttggggctgcctctggtgggtggaatgcctggcccccagactttctcacctctctttcctactcacaatccacatctctgtgacctctgccacaaggtctactccaaggacctcatctaaagtcatccttgctctgtcattctgttaccactcactgtcgcccaggctggagtgcagtggcgcgatctcagctcactgcaacctctgcctcctgggttcaagtgatccttctttctcagcctcccaagtagctgggactacaggcacaccagcacacccagctactttatttatttattggtagagatgaagtttcaccatgttgaccaggctggtctcgaactcctgacctcaagtgatccaccagcctcggcctcccaaagtgctgggattacaggcatgagccactgcgcccggccttcagcttaatttttaaagcactttttggttactgaaatgatattatttattgtttatctctccagtgtgtttcaggagagcaggcccttgtccgtctatttgccaccacatcccctggccgagattgggtctagaacaggttggcactcaataaatatttcttgaatactgggaaaacaacacaccagaaatggagcattccttgacgctgcgcttgcttctgagtctccacgttgctttttgtgcgaatctctgagtctgtctccggcttacctctccctctctatctctgtctctgtgtgtgtttctgctatctctgggacttctctgatttgtgcacctgtcagtctctcctcttcctcttctctctcctctgtatcaccttcctgtctttgactttttctctgtctgtgactctactagtttggtctctcctgctctccccctccctccccatcttgctcttcctcctgcctaccctcaacctcattctttctctctctctctctctctctctcgttctgtttggccttcagactctagaatccattctcccctaaccagttccctctccctcttccagcaaatatttgctgtctctcaattttttttttttttttgagacagagtctcgctctttcgcccaggctggagcgcagtggtgccatcacgggtcactgcagcctcaccctcccaggcccaagcgagatcctttcacctcagcctcctgagtagccgggactacaggcgtgcaccaccacacccggctaatttttgtatttttggtagagacaagatttcaatatgttggctggtctggaactcctgagctcaatctgcctgcctcagtctcccaaagtgctgggattaggagccacagcacccggccagatttgtctcttttaacacccgctccggcatccctcttctctccacgtatccgtctctctcactcagcgcttctccgtctcactgatttgtattccttttcctacatttcccagcatctcttcctgaaaccgccttggcagaattcttcctagggaccttcagtctctctcttcctggtccttccacacaggcctcggagagaaattctgaacacccagctctgatctgtacccttccgtcaagagaagggcacgcagagcccctggcagcatggcaccaccgctgccacgtcctcctcaagctgcgtctgtgcctgttttcccgccagactgggagccccttgagagcagggcaagatcaaaatcacctctccactcccagcaccgcccagcacaaggcttcgggggaggcctcaggaaacacttgctgagcaaatatggaagggaagcctactgggcgctgtcccctctgccttctcagtgaacttcaaacccatcccctccaatcaccgcacagcccttgcccccgcgcagctgtcatcctctctcaccatccttagaagagcctcagtccctctgcctggaactcaggcacctttttctctttttttctgagacaggatctcagtctgttgctcaggctggagtgtagtgccgcgatcctagctcactgcagcctcgaactcttggagtcaaatggtcctcctccctcagcctcctgagtagctgtgtccacaggtgtgctccaccacgcccggctaattttttttaatgttttgtagagacagggtttcgccatgttatccaggctggtctcaaactcctgggctcaagtgatactccagcctcagcctcccaaagcgctgggattacaggcatgagccaccgcgcccggccaccctggtacctttacactctagcttgtggctactttcccggcctcatctcccagccccaccttgtacatcagcatcccagaactgttagcactgaccccaatacatcatgctcgttcacttcctcccgttttcacccaagttgttctttggccccacaagcctttctcatgcctttcatcaaccagaagatgcccactcatttcttcaagacccagaatgggcatcatattctccaggaagcctaccccaagtgctgctcactcctggcagttggtcactctgtccaccgtgtgccacggtacccacggtggtccgggttccagcaccgattgccctgcctggatggcggtgtttgatgacaataaactgcttgagagcagggctagagtctgtttcacccctggggatctggatcctaacacacttcctggtaccttagcagatggccaaaaatggcaatgggtgagtggctgaatgaacgagtgacagacacatgagtctctaagccccacggctttctcctgcacaccagacaccatgactatgcttcagcatctgtgtaattacgtgcttcctcccacaagagtgtgagctccaagggcccgtgcccatgtttgatgctgtatttcagcacatctctgcctcctactcttgcctccgagttcctgtcttccctttgtacaccattcacgttagcgtcctgcttaaacccgttccacggccctcaccactcctagaataaaatctgaactcctgacctacgagcccctgcacaatctggccctgtctgtgtctccggcctcaccttgatccccgctcacctgcctcactacccttcagccctcgctgcaagctccttcctgccccggggcctttgcacgtgctgctctgcctgccacactcctgccccagctccgccctgctggcttcttctcatcctttcactgtccactgaaatctcttcctcacaactgggttaggctcccctgatggagcatttcatagcatctcgtttctcctatagcctaactgtaatttattgtgtatgtacatgatcgattaatgcctgtctcatgcacaagatgtttactctatgagacgtcggggcccctggctgttttcctgcctcctgcacgctgagcacggagcacaatgcctagctttttaaggcgcacaaataaattgccggtaatgaatgaatgaatgagaaggccctttctgtgcctcgttcgtgtcccctgctccaatgccttcttatgtaccagtgcctggtacacagtaggtgcttaataagcccttgtggaataatgaatgaaaaaaatgaatgaatgcccgcgtccaacccttctttctgcctttctgcatcccttcgctgtgtctctttatatagggcatatatatagtttgtgggtgtaactatgtattcgtgtattatgggcccctctccaggagttgggctgggctgggagtccctccctcccctccccccgccccgccccccatgcacacagcaaaacatgaaaaagaaaacatctcgaaactgcaaaaaacaccatggccctcccccctccccatagatcccccaaaaaaataaaacacgacgctccctcacagcggccccctccctcccctgccccctccctcggggtccctgcttcggagggggaggggggcggggagggtgggcgtggggcgggcccagcagtctccagcgcgctcacgggggaaagcgggggcgcccccgaccccggcagcctcgatgcacgcgcgcccgcgcacgcgccccggacacgcccctcggctcccccgccgcgcccctacacaggcgtggttttcctgttgagcgtgttggtgttggaggcggcggcctccttggccagggtcccgggggcgggcgcagagggcgcgggtggcgcgggcgcgggcggggcgggcggcccggtgaccgtgaccgtgacgccgccgcccgcctccttggggaaggcgttgtgcagcgtgaggaagccggacgcccccccgcggtcccgctcggcacccgccccgccgccgcctccgccgccgcccccggcgcccccggccgcgccgccgaacgcccccacggcgccgccgccgccgccgccggcccccgccagccccgcggccacgctgcccttggaggggtcgcggctgagcgtgtacatggagatgtccgtggaggcaaagcccgggcccccggggccgccgggagacgcgtcccgcgacggcgacggctcgctggagcgggagctagagcgggagcggcggcggtagcggaagcggtaactgggcagacggaggatggccgaggggccgctcccgccactgccgcccgcgcccccgccggccttgagcaggtccgagcgagactggcagtgcgcctcgcggctgcgctcgatgtagatgttgacggccagcacgcctatcacctcggccaggatgaacgacagcccgccgaagtagaaggaccagccgtacgagtagtggtttttcttctcctcgtcccgcttcgggcccggctcgcccgcgttggcggagatgtacacgatcacgccgatgatgttgctcaggcctgctgccacgaacaggatccctgcgcccagaatgatgttcctcttggacttgtagacgcgggaggccgccacgcacacacccccgagcagcagcaggatggcgctaaggatggggaagatgctggaggcccggacaactcggagtagatactccgcgctgtcgtggtcgtagtccgtgtcctccgggaaatgattgatcttcacgcagacgcctcttttcaacccttccaggcagcagatcctccagaggcccgagtgcgtgaggccgccggggtccttcttctccgaggcgccgccgcccccgcggtggggggtcccgtcgtcgccgccggccgtgaggttggtggtgttgcagatgagggcgcgcgtgtagagccagtagtcagtgctgatggcgatggtcatgaggccgaaggcggcgaaggcgcccaccgtcgtcagcagcacctgcacccccttctcgcaccagaggccccgctcttcgttccagcgcttcagcgactccagtttgaccacgggcagccggggggccgtgggccaccaccggggcagcgggggcggggccgtgccggcggctgggggggggttcacagcgcaggcagaagcggggggcccggggccggcggggctggggaggggggcggcgaggaggaggctgcggccggggagggggtcagagcgcggccatggtcggcggctggtggagggcaagg

SEQ ID NO: 16126 - RNA, 1514 nt, Homo sapiens
  source 1..1514: mol_type = other RNA
gctgggattacaggcatgagcccccacgcccagcccacacttttaattaatggagaattgaggctactaaacacatacttcaaggtatgaaaggaaatttgaaccactgttaagaattattctggagaataaaaggatctgaaggtggcatcaagagaatcacccatctccatatatgggagctactctagaaagaaatgcaaaaggtatatttcagtaatcttttcccaacttctctgttcccctgacaatactgagatcaacagaagcattggaaggtttcttttagataatagtgagagatacaggcagattgctagccaaatacagctctgggttactgtgataacacaggttccttcgaatgtatttattttcccaaattaaaaataagcagggatggaagtagttattatgcatttttcaaattctcctttcaacagtctatataaatgttgcagaatgctagactaggatgaaaagtaggagtcatgagaactgcagaagcctgagatcctaaaggaagtccgtaccatctgacttggcaatgtaagacacacacgttagtgtggggcacaaacgtggaatattaggagagagctggttccagcaccaaatccagagtcactcggggaaggaggtatggtggcaacactttatgcttaatattcaattctgctccagtagaacatggtacccaggagaacccaaaaagtccagcagagaatggcaaatccaaaccaggcaaccccccaggcgtgtcggttcattggaccagagatcagttcatagcagccctgattgtgataaaaaccaggcacgcctagtttacaagcctccaggttgagaggttctttaagattgttcataacacagcattgacgaggccagggatagtcagcatcattattctcagtccggaaggcagatgtgtatttttgccagtctgatggaccatttacgccacagcaattgtcctggagcatgagcctgtcccaggttttggtgactccattgtttttccactggtcatcattgtttggagggctgttgttttggtacctctctagcatctgcttcaggaagaggttgggtgtgaaaaagtcttgttgtgttgctgctgtgatacaagatgccacttcaaaggcatatactataaacatcagaatgaaatacgccagaagaattttcctgctggacttcatgatgcctacaatgcctagaacagacaggcagaagaggcagatgcccacaaatatgccgatccaggcagccccatagatgtcatcgttgtcggtggcttcaagcagtgggtagaggctgtgttggtcagatacaaagaagatgcactccgcagtcagggcaatgccgcaacaaccaataatcacatttccaaaaatcagcaggccctggaagcaacgaacagttgagttgtctttggccatcttcgggatttcccacaagctgaaggcaagcgcctcctctttctgcgcacacggtagggcccgctccgc

SEQ ID NO: 16127 - RNA, 1680 nt, Homo sapiens
  source 1..1680: mol_type = other RNA
gctgggattacaggcatgagcccccacgcctggcctgatcaagctgtttctcttgcttggaatgccctttgctgcctggccagctcctagtcatccttggaaacccagcttgaccatcccttcctttgaaagccttccttgtctctctggctcatgcgtctcctttggttcgtgcagtcagctgtgctctgtctgcataagcgtctctctcctgctcgtcccaggccttgcctccagccagcgtatagggcatgtactgagtgaagagggagactacatggcagccagggggagccagggtggggtccagcgaggaagggatgcagagctcaatcacaggcctgtgggaaggcaggccatccatggcatcttcaaaggcctgatgaaggaggagggtgtcttcacagttcaggtggatggagcattggtgatggggcagcggctggcccctgggagcattgggggccgccaggaagctgggcagcctgtctacggccacattgatcttggtgacaggcgaccgggtgtccagctgagagattctctccaggaactcctcaggaagccactcctgtggcgtcagcttcaggaaggtgatctgcggtgatgtgttggacagcaccattttgcttctcacctctgtgccatcttccagcacaactccttgaacacagccttcactgttcacctgcaccttcgccactgtcttttcagtgaagatgcttgctccatgtgtggtggctgagcttgcgatcgcatcagagagggcacccatgcccccctggacgtagccccaggccccctgcattccctccaggccccccatcacatggtgcagcagcacatacccactccccggagtgtggggacttgtcatggctccaatcactgcatctgtggctagagtggcttttaaaggctcagactcgaaccactgatccagcaccttggtaatgggagctgtgaggacctcataatatcggggaagctgggctcccaggatgcggcctgccttcagcaggggcttgagggtggagagcgacctcatcctttgcagcaaggagccatgctggaaggccgccatgtccacgggggccgcatccagcagagggtcaatggctaatgccaagcgatgcatgaactcctcatatttgggaaagacctgggcatccttctgggagaactgggcgatctgcttctggttttctgccatgtctgtgcccagcagaaggcacctgggcaccttgctgcctgcaccctcttccagcatgggggtgaaggagtaggggtttcgaagatgaagcctcagcccatgtttcttcagctccagatcagtgtaaatctgcggcctcagcaggctgagcaggtaggacgcgcgggagaacttaaaccctgggatgatctcctcagtgacagctgcacccccgatcacatggcgcctctcgaagacggcggtgttcacccccagtctctgcaggtacgctgcagccaccagtccgttgtgtcctgctcctatcaccaccgcatcatactcaggcttcagacctcccctggcttccgtgttatctcgtctccacgccgggaagggagaggcggccacagccttgcagagacctcggccacttgcagccatttctgccccaggctgggccttgctaggcagggagtttgctagcgatt

SEQ ID NO: 16128 - RNA, 1525 nt, Homo sapiens
  source 1..1525: mol_type = other RNA
gctgggattacaggcatgagcccccacgcctggcctgatcaagctgtttctcttgcttggaatgccctttgctgcctggccagctcctagtcatccttggaaacccagcttgaccatcccttcctttgaaagccttccttgtctctctggctcatgcgtctcctttggttcgtgcagtcagctgtgctgtgggaaggcaggccatccatggcatcttcaaaggcctgatgaaggaggagggtgtcttcacagttcaggtggatggagcattggtgatggggcagcggctggcccctgggagcattgggggccgccaggaagctgggcagcctgtctacggccacattgatcttggtgacaggcgaccgggtgtccagctgagagattctctccaggaactcctcaggaagccactcctgtggcgtcagcttcaggaaggtgatctgcggtgatgtgttggacagcaccattttgcttctcacctctgtgccatcttccagcacaactccttgaacacagccttcactgttcacctgcaccttcgccactgtcttttcagtgaagatgcttgctccatgtgtggtggctgagcttgcgatcgcatcagagagggcacccatgcccccctggacgtagccccaggccccctgcattccctccaggccccccatcacatggtgcagcagcacatacccactccccggagtgtggggacttgtcatggctccaatcactgcatctgtggctagagtggcttttaaaggctcagactcgaaccactgatccagcaccttggtaatgggagctgtgaggacctcataatatcggggaagctgggctcccaggatgcggcctgccttcagcaggggcttgagggtggagagcgacctcatcctttgcagcaaggagccatgctggaaggccgccatgtccacgggggccgcatccagcagagggtcaatggctaatgccaagcgatgcatgaactcctcatatttgggaaagacctgggcatccttctgggagaactgggcgatctgcttctggttttctgccatgtctgtgcccagcagaaggcacctgggcaccttgctgcctgcaccctcttccagcatgggggtgaaggagtaggggtttcgaagatgaagcctcagcccatgtttcttcagctccagatcagtgtaaatctgcggcctcagcaggctgagcaggtaggacgcgcgggagaacttaaaccctgggatgatctcctcagtgacagctgcacccccgatcacatggcgcctctcgaagacggcggtgttcacccccagtctctgcaggtacgctgcagccaccagtccgttgtgtcctgctcctatcaccaccgcatcatactcaggcttcagacctcccctggcttccgtgttatctcgtctccacgccgggaagggagaggcggccacagccttgcagagacctcggccacttgcagccatttctgccccaggctgggccttgctaggcagggagtttgctagcgatt

SEQ ID NO: 16129 - RNA, 7827 nt, Homo sapiens
  source 1..7827: mol_type = other RNA
gctgggattacaggcatgagcccccatgcctggcctatgcctggcttttaatagacactgaatacatgttttgagttaaccagaaatttaattattgaaattcaatagcattttgatatctactaattcctttttcagttatcccactcctcccttagaacctgtgtacatgatgctctctctgtctgggtttgtttcttccccagctagtcacatggctccctctctcacttcatatctgtactcaaacatcacctcttcacagaggccattcctaaccatctgttcaaatagccctcctacttctatcacactatatcctcttaccttgctttagacccattcttaatggatttaaaaatcattggtggagcatggtggctcgcgcctgtaatcccagcactttgggaggccgaggcgggcagatcatctgaggtcaggagttcaagaccagcctggccaacatggtaaaatcccatctctattaaaaatacaaaaattagctgggtgtggtggcagatgcctgtaatcccagctactcaggaggctgaggcaggagaatcgcttgaacctaggaggcaaaggttgcagtgagccaaaatcacgtcattgcactccagcctgggcaacaaaagcaagactctgtctcaaaaaaaaaaaaattatattcacaaaaaaatcccttagagttagggcaagtttttgtgctaaagtctctacaataaaatattattattattattattatttgagatggaatctcactctgtcacctaggctggagtgcagtggcgccatcttggctcactgaaacctctgcctcccaggttcaagtgattctcctgcctcagtctcccaagtagctgggattacaggcgcacatcaccacacctggctaatttttgtgtttttggtagagatggggtttcatcacgttgaccaggctggtctcgaactcctgacctcaggtgatctgcccaccttggcctcccaaagtgctgggattacaggtgtgagccaccgcacccagccaaaatcatgtttttaaaagaaagatttgaagatactttacaataaaagatataagaatgcagtaagcacacaaaaagatgcccagcatcactagtcatcagggaaattttcttttcttctttctttctttctttttttttttttttttgagacagtcttgctctgtcacccaggttggagtgcagtggcgcaattttggctcactgcatcctctgcctcctaggttcaagtgattctcgtgtctcagcctcccaagtagctgggactacaggtgtgtgccaccatgcctggctaatttttgtgtttttagtagagatggggtttccccatattggccaggctggtcttgaactcctgacctcaggtgatctacgcacctcagcctcccaaagtgctgggattacagacgtgagccaccacacctggcctggaaattttcaaaaggctaatactgctaagtgttggccaggatgtagaacaactggaacattcatacactgctgatgggagtacaaaatggtagagcgactttggaaagcactttggcagtttcttatacagttaaattttacacagaccatgcaacctaccaatctcgatcctaggtatctacccaagaaaaatggaaaacatacatacacatacatataaggacttgtacatgaatgttaatggcaacattattaataatagccaaaaactggtgacaaccaaatgtctatcaactgatgaatggataaacaaaatgtgatctattcatacagtggaatagtactcagcaatcaaaaggaaaaactactgatacatgctacagcatgaatgaatcttgcaaacatcattttaagtgaaagaaaccagactcggctgcaaactgtctgattccatctacatgacattctgaaatcagatcatcgttttctggaatcaggagcgtgggaaaggactgactataaattagcacaaggaaacattttaggatgatgaaaatatcttcagtgtggtagggacataactatatacaactgttaaaactcgtcaagcagtacacttaagacgggtgaattttttcatattcaagttctgcctcaataaagctgttccaagaatgttaaatatattgagagatatatgcacagaaaaggacgctatacttgtctcttgcggtaggattttgggtgcttttcattttcttgtctttgcttattgaaatcttgtaaaatttccacaatgattatgtagagcttttgtagagagagagaaaaacaacaataaaatgccatgatcataaataattgggttattcaacaaggaatgtattgttcattcaacattgttcattgtaatgaagcccatttagaccgcctccttctcatctatctttcatcagtgacacttctgaggggtgagctgaggaaacgggtgcaaaaaggtacagagcttaatagcaatcctttgtccatccagctctgggcttggctctcgccttgctttttggatgaatacacagtagactaatgataggggggctctcatcttcctttgccaacttcgccctccattccaatgcagatcagctcatgagtcctccaggccccaagagagactcctcagcacagggctgggcagactgtggtttgtggggtgcaggcccggcatccgcctccagctcacattggtctgttgggtgctgcctggtcttggtaaagtcaagaggccattcatcagtggagagccacaatgagggtgaccactcatgccgcacatggcaggacaggacacagagtccctccaggaggccctctgggtggggatgctcagtgtcaacaggcctctggcccttttcccccatcacgcatgccgttcatctccgaacttgccgcttatgaaagggcagtcaccttaggaaacccagccaacctggaggtggaggatggcgtgtcaggaatggtccacaccacttgcccgtgggcgcctaggctgcacaaggccccgtcagggtccaggtgtcagaacataggaatccagtgaggataataaatctataattataaaatagcttcataaaaacatcttgtagaggaaacatacaattttctagccactctagtcaggaagtaaagcccagcagaagcccagagcagctggggtgggcacagggaagtgagacacatcacagctgtcctggaagcctctgttttgtcagccataaagggtaagttgggagagaccctggttcccaacctggggtctctgtcctcaggattcacacaggcactattgtcaggaactacttctagcatctaaaaactccatacattattcacagtagccaaaagatagaaacaacctaagtgtccactgatggatgaatgaacaaaatgaggactatctagacaatgggatattattcagcttttaaaatgaaagaaattctgacacatgccacaacatggatgaaccttgaagacattgtgctaagtgaaagaagccagtcaaaaaggatagtattgtatgattcctcttgtatagaagtacctagagtggccaaattcacagacagaaagtagaatagtagttaccaggggctaggaggagaggggatgcggtgatattgtttatagatacagagttgcagtttgggataataaaaaattctgaaaatagatagtggtaatggttacacaacaatgtgaatatatttaattccagtcctgtacacttaaaaatggccaaaatggtaaattctatattatttatattttaccacatccacaaagaaacgaactccccacatacccacaatgtctcactgcttcattaaagcattgtcatgcctgttatcactcagatctgaatgggcaggtatagcctctgattgattttttagaagaaacaaaaataacagcaaaatatgttaattgtaaccttcagcgagagctgaaggagttttttgggcagttataacctttcaaagcatgacatcttttgggggaagacaaaggggctgtgatggaaaggttggcttgagtgagtactttggtatccctacccgcccccagcctcaaatgctgatcttgtacttggggaggctatgctaaaggagaaacacaccccagaggagacaccaggtggtgtcttcagacaattcccacccagccatagggataggcattttgggtttgagacggccctttctctggcttacttttagagcctggagtcagacttcttcacaacaaatagcccagaaccagctgggaactctctggcccatatgacacatgacactgatacagtaccagaaatgcatggcaccagctaataccactgaggggcaggagggcatactctctctcagaccctcatccatcacccccagaaccaggacaaggtcatgatggctcttggcagcctgctcagcaccagggcaagaacaactcaggctggacattacgagagtaaacacaatagatttctttcccagaccaagagcttgggcaccaggagtgggcattctggttcactgttaggcaaaaaagcctttggggaaattaccagctctcccgtcatccccaccttccttgaaaggcagcatgtggggtgggaagaacaatcagaagacaaattttaatctaaatcctgcccctctgtggccctggaaacttggcccctttgagcttcagtcactttgtgaaatgacaataacattcaatctccttcaacctcattactatggattaaatgagacggtgtctggggacatgcttggagaatgtattgtacaactgcttaggaattttcttctgcccctaaacctggaacttagagtggagcaaacagtaaacagtcactgtgtgtcggttaagggaacagagcctcagagccccgacccctggaaacgtttcttttttgtttactaaatttctagcaacaccgtgttttctacagaggtggggggaaatgtccatttaagtgcaagatgaaggggcctgtgaaaggaccctccaaggcaatcccatgtgctcccgtctcctggaaagaagccacatttcttcaagttgatgcaggggtgttgggggaaagccagagtaaacagggctctcctggtacctccttagagtacacaagtcatttgtgctggggaagagtttagtgtgtgtccttcaggagtctccaaatggcactccggctgcagcttcagttgaccaacttctccctcccaggaagcagggaggagagagaccttgggcaaggctttgtacctgcagccccagtgagcagatgtgtttcccaatgtggaaaatgcataccgtgcttccccttcctcgttgtctatgagtacgtaaaaggacacctcctgtggccctgcagcattacaatgtctgtggcattgtaagttcttgccttggtctgggagtccctcctctgttctctaagctcagacccagagggcaagacctagagtgccctgcaactgaggcagcctccccaaggctcgttctgaagctgccgtcctctgaggacaatggcttcttggaacttcttggaacaaacaagacaaaccaacacattagagccggcagcgggggcacaccgtgttcttctagaaaaggatcaaggggagtggcttcagtaacggaacatgagggactccctcacatggacacaaagcatcaagggacaggccggctttgcttttcgcttcttcctagctgcctaattaggacttactcagttcacagtgttctaccttaccgggccctcttggagccagctggagatgataaaaaccacacaggtattggagtcagatagcttcacatgccatttccacctgagaaacttgggtgagtcacatctctccaggcctcagtttttgcatctgtagaaggaagagaagacaacctatctccaaagcgttgtgacaattcagtgagatgatgtttgtcaagcccaccacacagggcaagttggttccttcccgtcccccgcatttgcctctactgagggtgaaggcagcagagaagacatcaccagcagctgcccaccactgcctggctctggagagggagggaccacgcatcctcacctaaccacaccaggccgctatcgcctgcatgtatctcgtgtccaatcggggccctgaggcagcgtcccgccctccctggaccccctcagatatcccaggctggaatggtgaggggcaggtgggagcagccaggcccttccctgggcaagccgtggtgagccacccgcccattccgcagcgggaggcggccgggcctgggggccccactgctagggcccgactcagagggcagcccggagtcgctgggccgcaccaccacgaagacccgcctgtgcagaagcccgccgggccgctcggagtaggcctccttgtggctccccgacgggcgcgggcagaggcgggcgcggaaggcggcctggaagccgcggcggaagttctcgttgaagtagccgtagatgatggggttggcgctgctgttgaagaaggccagccagtgcgcgaaggggaaggcgtagacggtgaccaggtgcagctgcggcgcgctgagctgcccgtagtcgatgagcagcagcagcgcccagagcggcagccaggacagcgtgaagaacagcgccaccatgaccagcatgtgcaccacgcgcgctctgcgccgcgatgctcgcgggtccgcagcctcctcgcccccgggggccgggcccggggcctggcagagcttgcgcgcgatgcgggcgtacatgaccacgatgagcgccagcggcgccaggtagatgtgcgagaagagcacagtggtgtagaccctgcgcatgcccttctcgggccaggcctcccagcaggagtagagcgggtaggagcggttgcgggcgtccaccatgaagtggtgctcctcacgggtgacggtcagcgtgacggccgagggacacatgatgagcagcgccagggcccagatgacggcgatggtgacgagcgccttccgcagggtcagcttctcgcggaaagggtgcacgatgcagcggaacctttccacagcaatggccaccagtgtgaaaacggaagccgacacagacatgccctgcaccaagccgctcatcttgcatgtggcattgtcgaagggccacccagtgatgaggttgtccacaagggtggtgggcatgcagaagatgcccaccagcaggtcactgacagccaggttgaggatgaacatgttggtgacagtatgcatgtgccggttcttgagcacgatgaaacagaccagggtgttgcccaccatgcagagcaggaagatgagcgcataggccacaatgaacatggccgccacaggggaggtgtgctgatagtaggaggagaaggtgaggtttgtagccggggtggcctcagtgttagtcccattctgacttaggggccaactgctgttgggaggctgggagggctccccctccatgatgcccccagttgcgggctccggcggtctccgatggcgggaggcagcgggccccttcgggccagcgggcagagggacggtctccgggcacttggttgcgggctgcgcccctgcctccgcgctccgcaggtccggtcggtccgggcagaggtgagcagggggcgtgcgctcccaggccccgggccctggccggtttccctcccctcgggctgactggctcccgcgcagcgctgctgcccgcagggctcagccgcccgccgcccctcgcctcccgaccaggggaaggagggggctcgtgaggcgcagtcgtcatggcacccgcgcacct

SEQ ID NO: 16130 - RNA, 2451 nt, Homo sapiens
  source 1..2451: mol_type = other RNA
gctgggattacaggcatgagcccccgtgcccaaactgtttattaaattaaaacttgtgccacaccaggtttcctcaaagaacctctgggtccacagtgggtggggctgccatgcggttggtgccctggggcaaagcacagaactgcctcctgcacaaggccacggcccctgcagccagccgcaacttcggctctctcctggccccacgaagccccagagtcccctccccgctggcccctgcccccaatgcaggctctgcctgtcacttgctggacgagttccccagcgttcctcagcgtctcaaacatcaaaggcttcatttgaaaatgggataaaaacatctccagggcggggcggctgctaacagcagaggcctccatgggagacgctggtacagccaattccaggcgccacgtacttcaagcacccagagaactgcggccagttattttttctgattttatattatttcttaaatagggcgtctcgcttgttgcccaggctggtcttgaactcctgggcaaagtgatcgtcctgccttggcctaccaaatgctgggatcccaggcgtgagcccctgcgcccagctgactgaggcctgctctaacttcatgtgacggagcgagtttcctggcttggaaataactgaaaagattcattttctctttgtgtacaaaggattcaaaatattttcacatcttccttctgccagttaaacgtgccgtggctccaatacacaccaaagccaagcgtacttggctgcctcaggaaggctgggaggaagtgccagatggtatcagcgacagcggtggggaccgggcggggacgggccagctctgtcctcccaacacggcaccaggcactcggcctcatgggggaggcccggccagcgggaggcagccacaagtccaggccacgtgggaggtgagcgtggggggagcagtgcctgccccacctccaccactgctcagaagccgcagcagtcatgaccaagaggaccgggtgccctggtgcccacaccctgggcctcgaacctgcggcgtgcacgtgggtgccaggaaagggacagcgggggacagactgtggccctgggcagcgatgccccacaaaggagtcccatccaggctggaggacgtggctcctggccacaggggctccggcctctcctcccggattccagtcagggttcccatgacacccggacaaaccccaggtgaaacgccctcgcagccctgtcagagcagcccggggccagggctcttcatcacgcggtgctgaagcagctccaggctggggcggcctccagggagggcagggagtcagggccccaggagccctggtgcacccgaggactccgctgcccgccggggcccgggggaagcagcacttactggtcctcgttgcggaagacgccccacaccacgctgacggccacgcagaagagcgccaggagcagcatacgggcctgcgggcgctgcacttgccgaagggcagccgccgcacacagggcgccaggcagctgtagaggccggtggcggaggccaggcagaagatcccgatgaccacgtacacgaggagatcgtagaaatagtagagcagcaccagcatggagcagcacatcaccacaaacacgcaggtcatcaccggcgtcacgtccaccgcctcgtcctcctgcttctcgggcccatcgtcgcgcttgtgcttcatgtaccttttcttcacgtcccgactcccggcccagtagccgccgatggcgacggtgcccacagccatgatgaagatgatgaccatgttgtagtccagcaccggctccttaggcgcatacagcgccgccctcaccgtgcggccgaaacgcgtgaagatgtccagcatgtctttgtagctgagcagggccacgggaatgccaatctcatcatactgcgtcttattaccccccggggggaccagcctctccctgctgacgatgagcagcccgcgtgctccgctgccctgggccagcctcactttctcatagaaggtgcagttcccccgcgccaccagcgggatctggttgctgaagccacgggcggggaggtcggctgcggagcagagcagggaggccgtccagttgcgcagctgcaggaaagatgccttgctgaggtcgtgcggaagatgggcccactgcgggttgtagaggatgcagtagtctttgccttcggggcccccggcctgggagaccacgtgcaccatgccgtactcacaggccacctgggccgcgaggagcagaaaggccgccaaaagccgcgccagcgcagccgccaccgctgccgccatgtcggccggtgcccgccgcaaccaacggcagatgtttcccagcaacgccccgagaccccgggccacgcatgcgccgcgcatgcgcgtgggggaggtcaaagggcgcggggcggtgcctgcgaagagccacacggcgcga

SEQ ID NO: 16131 - RNA, 307 nt, Homo sapiens
  source 1..307: mol_type = other RNA
gctgggattacaggcatgagcccccttgtccatccgcacaccacacccacttctgaagagcacctgggtagactggccccctcccacaactctggccctctccgtggctgcagggagctttgccgaagtggggatgtgagccacccttgggatgggggacagagaccccaccccactcccctgccctgtccccacccccatgaggaccaccaccaaaggtctagttgaaagagagtgacatcggtggggcgcggtggctcacacctgtaatcccagcactttgaaaagttcgaggcgggcggatcgc

SEQ ID NO: 16132 - RNA, 688 nt, Homo sapiens
  source 1..688: mol_type = other RNA
gctgggattacaggcatgagcccccttgtccatccgcacaccacacccacttctgaagagcacctgggtagactggccccctcccacaactctggccctctccgtggctgcagggagctttgccgaagtggggatgtgagccacccttgggatgggggacagagaccccaccccactcccctgccctgtccccacccccatgaggaccaccaccaaaggtctagttgaaagagagtgacatcggtggggcgcggtggctcacacctgtaatcccagcactttgaaaagttcgaggcgggcggatcgcctgaggtcaggagttcgagaccagcctggccaacatggggaaacgctgtctctactaaaaatacaacaattagccaggcgtggtggtgcgtgcctgtagtcccagctactcaggaggctgaggcaggagaatcacttgaaccggggaggcggaggttgcggtgagtggagattgcgccactgcactccagcctgcgtggcagagcaagactccatctcaaaaaaaataaagagggtgaaacagggatagaagcatgacagacccgtcacctccctgcccatacataccaggtggcccgctgggtaaggtggtgatccctgggagcagggccagcagcagcacggtgcccagcatgctggaccagctgaggtcggagtgttt

SEQ ID NO: 16133 - RNA, 902 nt, Homo sapiens
  source 1..902: mol_type = other RNA
gctgggattacaggcatgagcccctgcccctggcccttaaaatattttactaaaactaagtaggcatatatatgtctgcagtcagtgtcttgctttgcattccccagaacagatgctgagtcaaggatccagtgaaagtacttcctttgggaaatgatcccaggaagcactcacaggggagtggggaagtgagatggtaaggaaaggcaagccacaaatagctcattatcaggcaggttactactgtgggaatggagttagaggccgcaggggaaccctgggagccagtataggacacacgctgcagagttttcctcactgagggttgagggcgtgggatatttatatgccagtcacttacccctgcttgtgtcttgctggggagtggggaatgatcattttcaagtcctatgacagtaggcaaaatggactctttaggccagagaaagccctttttggatgctttcctctctttattaaaatcttgcgcagtgtcttttcattttttcttcagaggtaattcagtctgttcttaccggtttcctgaaatgaaagcatcttatgttgccgtagcatgtttatcaccactaagaagctaacatcattgtgaattattaactaaacttcagattttatttggatttccccaggtttttcattagtatctttgttctgttcaggatacagtccaggacactacattgcattaaacagattctctttgaattgagagatagcatgtgctccatgtggttctgcatttagtgttctcaactgatgatgtcataattcattgatttcaaaatccaatggaatgtaactattatttttgagtacttcttctcctttttttttttttaaacggagtttcactcttgttgcccaggctggagtgcaatggc

SEQ ID NO: 16134 - RNA, 862 nt, Homo sapiens
  source 1..862: mol_type = other RNA
gctgggattacaggcatgagcccctgcccctggcccttaaaatattttactaaaactaagtaggcatatatatgtctgcagtcagtgtcttgctttgcattccccagaacagatgctgagtcaaggatccagtgaaagtacttcctttgggaaatgatcccaggaagcactcacaggggagtggggaagtgagatggtaaggaaaggcaagccacaaatagctcattatcaggcaggttactactgtgggaatggagttagaggccgcaggggaaccctgggagccagtataggacacacgctgcagagttttcctcactgagggttgagggcgtgggatatttatatgccagtcacttacccctgcttgtgtcttgctggggagtggggaatgatcattttcaagtcctatgacagtaggcaaaatggactctttaggccagagaaagccctttttggatgctttcctctctttattaaaatcttgcgcagtgtcttttcattttttcttcagaggtaattcagtctgttcttagtaattcttttttgcagaggtgctgtgcttcagcagggaactgtgcttgttgtgactgcttggggacatgggctgatgagcagcatcttctcagtattgctggtccctgtgcagagggaaaagagctgtggaaggtctggaattaacatttagatgcctttttccactcatagctcacaggccagaagtaatcaaatggttccatccaacaggccagaaatatttggtgaacagcactaatgactaccacagttagtttttgttttgttttgtttttgtttttgtttttgtttttgagactgagtctcgctctgtcgtccaggctgg

SEQ ID NO: 16135 - RNA, 2108 nt, Homo sapiens
  source 1..2108: mol_type = other RNA
gctgggattacaggcatgagcccctgtgcccagcctcagtcagctttcacagtctaactttgtgccaagaagttagtaagatctgaaactagtcaaagtagcttccatttattcacagttttaaaaacatttttcaagtttagtcaacttcccaatataatcaaaggacaaaatggcaataaaaaatatacttcatcagatcttagagttatacaatcagttaaaaaatagatattgggttttaaacaactgacatatgctttccttttccccctttaaaggttttcagtagtctatctgaaatcactgaatcacttttcttctcctccacagaattcagaactttttcacccggaactggagaaggagcactccgtcattagctgaggggaatggcaaggatccaggggtcctccatgactacacaaccatcctcctgagcacctttaggaaatccaatgctgtctgagaagcagcagggccagatccagatctatggaaaattaatatctgcagtgcttcctgaaggtcacctcagtctttatgccatttcaaaagctagcccggggcttgagaagaaaagggaagtggcattccagccatatttggggtgcaatttaattttcattgcgtacctcatgaacaggggcaataacacattctaggatattcttccagcccacccactcttcctctttctcttcttctctttctctaacgagtggtagtgacaggatgcaagtctgcgctcttggtagataaacggagaagcaggagaaagaactattccataatcagttaaacggggagttttcagaatcctgtcttgtcatttaagtgacttactgaagtcctactaagttattgagactatatttctttactttttgcactgggacattgaagcattgagacaccagaagtccaaaagacgaaaaatgtgaaaatcacaaatttaaagaaaatgtagaggtctcagttctgaaacaccatgcttcaagtgttgtcatttttgagaacatttttaaaaggcatctaatattccaggacatacggttcccattactggcccagcaggtacacagggtctcccactttgatggtccctgggttttccagcacaaaatactgcccaaagagtggtgattttccatataactttcgttctgaagggtcacactggcgataactcttcagtgtttccagcggttccttcctgctcatgacaccggtgtctgggtccactgtggttaaaatgcatctggaacaagccatcacccttttcagttccacgtcaccaataagaagctcatcccaagaatcctctgcatagacatcgcatcctgaaattacaatattgggcctgaagttggttgctttaactttcttctctagcctggagttgagatccgccagcgacgcctcagaaaggatcaagaatgggctggtgtctgagtaagcaatctggtccttgggtcggaacaagtctgctatttgatgaggacgtctcggtcgcatgtgaggctcgaagtgcaccaggcggtagggctgtgacttcaggaagctggttatccactgggcggtggcctcgccacagtccctgccctctatctccaggccgtgcactctgcacttgtgcactgcatttgtggtgggcgttttgataggcagtagtaggtcctttgtgtaggctgcactgagagtcagggtgtcaccatcgcaggtcagggaaatcaggaccaggcgaggttcctggcgagcagtaaccatgtttccctcctggttgatcacaagccaaaacctgtcccgcaggttgccgctgcgcagccccatggccgtgcactccgcctcgctcaccggcacccccttgcaggatttcacagggtagatccagagctgcgccactgtgcccacctgctgcagcagccgccggcgccgcgtgggccatgcgcggcgccaggcgacagcccccagcgccaccgcggtcaggcccagcgcggcaaccccgagccacccgggccgggattgcgcgaggaggacaaagcgcgccagcgcggaggagccggcggcgcccatggctggcttctccgcgaggtggcggcggcaag

SEQ ID NO: 16136 - RNA, 2132 nt, Homo sapiens
  source 1..2132: mol_type = other RNA
gctgggattacaggcatgagcccggcaccccgccaaatctctggcatcttttcttcttcttcttcttttttttttttttttgagatggaatttcaatcttcttgcccgggctggagtgcaatggcaccatctcggctcactgcaacctccacctctccagttcaagcgattctcctgcctcagcctccctagtagctgggattacaggtgcacgccaccacacccagctaatttttgtatttttagtagagacagggtttcactatgttggccaggctggtctcaaactcctgacctcaggcaacccaccagcctcagcctcccaaagtgctgggattacaggcatgagccccacgcacggccaaatctctggttatcttttctaacctctaaattcacattcccttggtttagtgtttactgctcttatgaagtgagagaaaccccacttggcaaaagcacgttggtatttcctagagaggctctgggttttgcttttgtttttgtttttgtttttttaagttgttgtttgtttgtttttactttcatctgttttaaagtttccatggtagcatggtagattgtggtctattgagcagtcagaaagcctgggtttgatttctggtctgcactaacctgctatgtgctcctgtgcattccgatttacctcactgaggccgtttcttcatgaggagaaactcaatgaggaaatttgtgttaaatcagattatcaagagttgcagtattatataaagccaacggaagcaaggctgttttggttggatttgaagaggaaccatggacgcacatcctttcttgcccatctgcatggcctgagaataaccttcatatcctctccaaggaactctaggattcctatgtagaaagtagccagaaaatgatcagtcctgatggtttcgaagatctcaaactgtaccattcaatagttctatacctggcagaaggtcagtgcatctctcccttgcagccagtcccgggaaacaggtctctgaaagaatggaagcctttcaaattctttttttatggagatggctggcagccaaaggagcaggattatagagaccccaaactagactgaagggattgagggacaaatgagaaaggggaatgtcaaggcaaattttcacaatggcttgcactattccaagtaacaggaactaatttatctcagaaacaccgggcttactgctaaaaccaacactgctttctagctcgttcctaataacacccatttctgggctttctaacatcctatttggtcattaatagcagccttcacagaaacataaatgaaactaagaattgaatatttatatttatgatgtaaaataaaattactttcccaagtgtttcagccaagtgttgacaggaaataaaacagaattcacagggatagtggattttctgacaagtttgagatgtcagcatcgcacgctttcaggcaaagtgcaacagaaggaactgtacttgtcattacaccaactgcctccttcccagtggagggtctttgatcctggtactatgactcactgggtcactaaggacttcagttgtccctccaccatggtgggtcttgggtttctccattcagtccagataacacatgtaaaggatctgaggtccctagataagaagcaacattcagtagaatttggcattcataggatgatgaaatttatgacatcattatcccagttctcacggttataatccacagaaagcttctctttattctcagaactagcccttgtagtggccttgaatgtgcaaacgttaccctttagtaatgtttgaggcagaatttgaaaatctgaaacatgattcaaagctaccctacaataactaagctgccatagttacctaaggctgcttcccaatatgttttctatgaatctgcctttccaatagagcacagtgcagggaaaaggggagggggcaattgtacaaaagacacaaaaggtccagttttagtttggcccatgactgccatgccctggaattctgtacagtctcagaaagagagtgtcactgattattaaaaatacataatttcttcttttttatttttttaatttttagaaacatgggtcttactatgttgcccaggatag

SEQ ID NO: 16137 - RNA, 3930 nt, Homo sapiens
  source 1..3930: mol_type = other RNA
gctgggattacaggcatgagcccggcaccccgccaaatctctggcatcttttcttcttcttcttcttttttttttttttttgagatggaatttcaatcttcttgcccgggctggagtgcaatggcaccatctcggctcactgcaacctccacctctccagttcaagcgattctcctgcctcagcctccctagtagctgggattacaggtgcacgccaccacacccagctaatttttgtatttttagtagagacagggtttcactatgttggccaggctggtctcaaactcctgacctcaggcaacccaccagcctcagcctcccaaagtgctgggattacaggcatgagccccacgcacggccaaatctctggttatcttttctaacctctaaattcacattcccttggtttagtgtttactgctcttatgaagtgagagaaaccccacttggcaaaagcacgttggtatttcctagagaggctctgggttttgcttttgtttttgtttttgtttttttaagttgttgtttgtttgtttttactttcatctgttttaaagtttccatggtagcatggtagattgtggtctattgagcagtcagaaagcctgggtttgatttctggtctgcactaacctgctatgtgctcctgtgcattccgatttacctcactgaggccgtttcttcatgaggagaaactcaatgaggaaatttgtgttaaatcagattatcaagagttgcagtattatataaagccaacggaagcaaggctgttttggttggatttgaagaggaaccatggacgcacatcctttcttgcccatctgcatggcctgagaataaccttcatatcctctccaaggaactctaggattcctatgtagaaagtagccagaaaatgatcagtcctgatggtttcgaagatctcaaactgtaccattcaatagttctatacctggcagaaggtcagtgcatctctcccttgctgatggttattcattcaaacatgaaaggagaaaataactggtttagtctttctcaggaacacacactctttttttagagtcagactattttcttcttcaatgagttaagttttactagagacacttagtagtatatttggaaacttaaaatgtaatagtagtacctcttcttttctgatcttctgtttattcccttacctacctaaaaagatcaatcacttactaggattaacccaacacttaggctcaatcaactgcatgaacgtgtttggactctcaaaatactatatttcctcaattttacaacatactttttttaaacatttaaaaatttctaatataatcattagtttaaatttttacgtaaaaagcctcaaatgccagggagtgaagagaggtggttctcattgcctgtgcatttgcaagcttagaaatgtctaaaggaaaggtatcttttcattcttcctcccaatcctttcattcatctaacaaactgttgttcactgagtgcctgttttgtatcacgtacatttctgggcacagggagtacagagtacaatgataggcaagcatcaatgatagactctcaaagagtctcattctagtagggaaaggtagatgataaacaattgaactgataaataaagaattttcaattgtgataaatgttacaaagaaagcaagacagaaagatcaggaagtggggtaagtcagggaggtttctctgattaaataacatgtaagcagaaagctgagtgctgagcagttgcaagggcagtccctgtagagaaaacagtaagtgcaggggccctggggcaagctggcctgagctcagcagaataagggaacatggagacaccctgttgactcatttacatggctagctgaacaagaagttccatttaacttaaatttggatttctatctcttaaacaaaatatctttcaaaagatacattatgatgctagactaaagctaacagagaaaaacgcagaactaaagtccattgtttctggtaaagcaatggcccgtttggtccccatatagagataaagctgtttaaatgcatcatggaaaaataggcccactctcatgatgaaaggcttatagggagccaaattcctttccaaagctgttattaaacagagcatctttttttttttctttttaatggttgcagcacaccaacatggcacaggtatacatatgtaacaaacctgcacgttgtgcacatttaccctagaacttaaagtatgataaaaaaaaaaaatgaaaagagcatcttaaaggactatctctatttccagcagaccttcaagagaagtttaaaggaatatgtaatgttatagtcaattctaaattactaaaaaggccagaagaggcagattactgcaaacagcctatctgagcactgcagtacacaattgtcaaggatcaaaatcagctcagaggaatcataaaactccaagaagccttcgaatcaaacatgaatggtgacagtgaagaagaaagagaaatgtcatcacatcaataaacataggctaagtgagtaaaggaagaaacgtgtgtacatttcctacaataaggttgttcccctcccaatcttgttattaaatccatagtgtgtcttacaaacatggactctcagaatcatagaaataccacagctctttctccagcctgctaaagtgcttggaatttccaccattaagctctaggaagttctgtaagaacattttatcaagaaatataacacagtaacacatcacaatctgtttgaaaaatgagcatgatttatcttaccagccagtcccgggaaacaggtctctgaaagaatggaagcctttcaaattctttttttatggagatggctggcagccaaaggagcaggattatagagaccccaaactagactgaagggattgagggacaaatgagaaaggggaatgtcaaggcaaattttcacaatggcttgcactattccaagtaacaggaactaatttatctcagaaacaccgggcttactgctaaaaccaacactgctttctagctcgttcctaataacacccatttctgggctttctaacatcctatttggtcattaatagcagccttcacagaaacataaatgaaactaagaattgaatatttatatttatgatgtaaaataaaattactttcccaagtgtttcagccaagtgttgacaggaaataaaacagaattcacagggatagtggattttctgacaagtttgagatgtcagcatcgcacgctttcaggcaaagtgcaacagaaggaactgtacttgtcattacaccaactgcctccttcccagtggagggtctttgatcctggtactatgactcactgggtcactaaggacttcagttgtccctccaccatggtgggtcttgggtttctccattcagtccagataacacatgtaaaggatctgaggtccctagataagaagcaacattcagtagaatttggcattcataggatgatgaaatttatgacatcattatcccagttctcacggttataatccacagaaagcttctctttattctcagaactagcccttgtagtggccttgaatgtgcaaacgttaccctttagtaatgtttgaggcagaatttgaaaatctgaaacatgattcaaagctaccctacaataactaagctgccatagttacctaaggctgcttcccaatatgttttctatgaatctgcctttccaatagagcacagtgcagggaaaaggggagggggcaattgtacaaaagacacaaaaggtccagttttagtttggcccatgactgccatgccctggaattctgtacagtctcagaaagagagtgtcactgattattaaaaatacataatttcttcttttttatttttttaatttttagaaacatgggtcttactatgttgccca

SEQ ID NO: 16138 - RNA, 2027 nt, Homo sapiens
  source 1..2027: mol_type = other RNA
gctgggattacaggcatgagccgcagtgcctggcttatgtgtgatcttttaaaggactgtctattaccaatccaaagttactatatttttcattgcaacaatttggggtcttattcttattgtaggtgctttaaactcattacaccagagtgttattctacccaaagtttgtgacccagctcaggataactgtgagaagcaatttagtgtagtgttgcttaacttgcccaccgaagtggacaagttaaatttccctgtgactcagtcaccttcttggtaaatgataacaattatttcttcctcacagagttgtaatgatgattaaataagactgtgcttgataagcacttcaaacagtggttatcagagagtaatcactgaagtgttaattattatatagttaataattatattataatcttttttattttgtccattattttttcttcctgggaagggacatgcagaaaggtatacatgtttaatatataatcatcttggttttttttctccaaccattaaatattttgctcaaaggccctatactagttttagtttcaatcattcttctggaaacctacagggtaacacatccgtagctcttcaatttatttcctcaaggtggggtttaatttttccctagcttatcccactaatcataccatagtcatgccctctctgacttttgcctctaatcaatgtctacctacaggacttacttgcacgtagtcttcttcatactccattggctttcgtttttttcttgctttccccttgattttcttcttgtttgttccttgctctttccctccaaggattgcaaagtctcatcccattgcagtgtgagctcaatatccaaaatcttgtcatctaaatcaggtccaggtgcagttggggctcctcagttttaattccttaagtacagctctttgagtacatttcttcttcttaacctgtgaaaccttaatttatttaaagcgctcctatgtgactgaatcgtattctgaggcaccatctttgtttcttctgaggtcttcacgaatggttttaagtcacacccttgatttcatctttaatcttccttctctcaattcaacgccttcctgtaagacccaagaagaaatcaggtgtcaccttcaacactatttgaaaatctccttagctagattacccttgccaatagacacattttccatataatttcagaaaactgtattgctaaactttctaccactgcataacaaagagcccctttcctttagtttccaataagatttttctttcttcaagccctcaccttccatgtcttcaaagtccaaaatttcatagtgttgttcaagcgcattcttcatcaatcactttacttttgacacatttcagagtagtttgcaaaatcagtacactcactccagatacttcagcatgcatatcactgactaatgtttaatatttatcttaaagtatgtatattttcttttgaggtaaagttaatatacaataaatgtacaaatgtcaaatataccattcaatgaattttgacaaataaatacaactatgtaattcaaagcccagtctggattgaaaaaacaggatcatcacccccagaatcctttcatgccacctgggtcaatcacgatgctaaattccttgcctcagaggcaacaactgttccgatattttttctaaaaaattaattttgcctattctaaaatggcatataaatggaatcatacagttacatgctgttttgtttaaggcttctttcattcgacacagtattatttagattcctccatgtcagtgtatagtatttcacttctttttatcgctgagcacattaagtctgctagggctgccataacaaaatgccatagacagggtggctgaaacaacagttctaaaagctagaagtctgcgatcaagatgtctacaggtgtggtttctcctgaggcctctccccttcacttgcagatggccttctcactatgtcttcacatggtcttttctctgtctgtgcatatccctgg

SEQ ID NO: 16139 - RNA, 2331 nt, Homo sapiens
  source 1..2331: mol_type = other RNA
gctgggattacaggcatgagccgcagtgcctggcttatgtgtgatcttttaaaggactgtctattaccaatccaaagttactatatttttcattgcaacaatttggggtcttattcttattgtaggtgctttaaactcattacaccagagtgttattctacccaaagtttgtgacccagctcaggataactgtgagaagcaatttagtgtagtgttgcttaacttgcccaccgaagtggacaagttaaatttccctgtgactcagtcaccttcttggtaaatgataacaattatttcttcctcacagagttgtaatgatgattaaataagactgtgcttgataagcacttcaaacagtggttatcagagagtaatcactgaagtgttaattattatatagttaataattatattataatcttttttattttgtccattattttttcttcctgggaagggacatgcagaaaggtatacatgtttaatatataatcatcttggttttttttctccaaccattaaatattttgctcaaaggccctatactagttttagtttcaatcattcttctggaaacctacagggtaacacatccgtagctcttcaatttatttcctcaaggtggggtttaatttttccctagcttatcccactaatcataccatagtcatgccctctctgacttttgcctctaatcaatgtctacctacaggacttacttgcacgtagtcttcttcatactccattggctttcgtttttttcttgctttccccttgattttcttcttgtttgttccttgctctttctggactcattggtaaaacaataaagaccttttattgagcagttaatactgttactgtataaggcacactgtaacataatcctcacggcatccctaggaggtaggtggtacccactttacaaagaaccagaggctcagagagatgggttctgggggtcatggcccatctgcttggctgtgagccagactccaaggatactgttgctttcactttcctttttacctgtcctctctctttcagctcaggaaaattggattaaccgtgttctcatgtgttttgttggtcacatgccattgctattttccctccaaggattgcaaagtctcatcccattgcagtgtgagctcaatatccaaaatcttgtcatctaaatcaggtccaggtgcagttggggctcctcagttttaattccttaagtacagctctttgagtacatttcttcttcttaacctgtgaaaccttaatttatttaaagcgctcctatgtgactgaatcgtattctgaggcaccatctttgtttcttctgaggtcttcacgaatggttttaagtcacacccttgatttcatctttaatcttccttctctcaattcaacgccttcctgtaagacccaagaagaaatcaggtgtcaccttcaacactatttgaaaatctccttagctagattacccttgccaatagacacattttccatataatttcagaaaactgtattgctaaactttctaccactgcataacaaagagcccctttcctttagtttccaataagatttttctttcttcaagccctcaccttccatgtcttcaaagtccaaaatttcatagtgttgttcaagcgcattcttcatcaatcactttacttttgacacatttcagagtagtttgcaaaatcagtacactcactccagatacttcagcatgcatatcactgactaatgtttaatatttatcttaaagtatgtatattttcttttgaggtaaagttaatatacaataaatgtacaaatgtcaaatataccattcaatgaattttgacaaataaatacaactatgtaattcaaagcccagtctggattgaaaaaacaggatcatcacccccagaatcctttcatgccacctgggtcaatcacgatgctaaattccttgcctcagaggcaacaactgttccgatattttttctaaaaaattaattttgcctattctaaaatggcatataaatggaatcatacagttacatgctgttttgtttaaggcttctttcattcgacacagtattatttagattcctccatgtcagtgtatagtatttcacttctttttatcgctgagcacattaagtctgctagggctgccataacaaaatgccatagacagggtggctgaaacaacagttctaaaagctagaagtctgcgatcaagatgtctacaggtgtggtttctcctgaggcctctccccttcacttgcagatggccttctcactatgtcttcacatggtcttttctctgtctgtgcatatccctgg

SEQ ID NO: 16140 - RNA, 3305 nt, Homo sapiens
  source 1..3305: mol_type = other RNA
gctgggattacaggcatgagccgcagtgcctggcttatgtgtgatcttttaaaggactgtctattaccaatccaaagttactatatttttcattgcaacaatttggggtcttattcttattgtaggtgctttaaactcattacaccagagtgttattctacccaaagtttgtgacccagctcaggataactgtgagaagcaatttagtgtagtgttgcttaacttgcccaccgaagtggacaagttaaatttccctgtgactcagtcaccttcttggtaaatgataacaattatttcttcctcacagagttgtaatgatgattaaataagactgtgcttgataagcacttcaaacagtggttatcagagagtaatcactgaagtgttaattattatatagttaataattatattataatcttttttattttgtccattattttttcttcctgggaagggacatgcagaaaggtatacatgtttaatatataatcatcttggttttttttctccaaccattaaatattttgctcaaaggccctatactagttttagtttcaatcattcttctggaaacctacagggtaacacatccgtagctcttcaatttatttcctcaaggtggggtttaatttttccctagcttatcccactaatcataccatagtcatgccctctctgacttttgcctctaatcaatgtctacctacaggacttacttgcacgtagtcttcttcatactccattggctttcgtttttttcttgctttccccttgattttcttcttgtttgttccttgctctttctggactcattggtaaaacaataaagaccttttattgagcagttaatactgttactgtataaggcacactgtaacataatcctcacggcatccctaggaggtaggtggtacccactttacaaagaaccagaggctcagagagatgggttctgggggtcatggcccatctgcttggctgtgagccagactccaaggatactgttgctttcactttcctttttacctgtcctctctctttcagctcaggaaaattggattaaccgtgttctcatgtgttttgttggtcacatgccattgctattttttgtcaggcatactgtctgtcctttcaggagtccttctctaattgtttacacgcatagaacttgagtctccagctggttcgtaagtcccttggggccagggtttcttttgtgtccactatagtacctaacacagtttggggctcttatttggcagatatgaccagatgtatgttttctaaatataactgcattttttctggatcaattttttaaaaatgttatgctatatttaaattttagatttgtttcaactttgcttaagactgtactattccttcagtttttctttatgcttgtacaggaactacttggcatgatgctgtcagctgtaatatacatttaggctttaatatcaccaggcaagagcatctgtcaagatagatgatgttccctcctttgccatagctgggcctcacatttctgtcgctgaatacatgcctctagtttgttcagtattttaagcagcagatttataactttaaagtttttaaatccatgcaactacctcatctctagcaaccatttcacatctaaataatcatccttggcctgcttaataatgtgagtataaagatttgccaatagttctttttcccccagtaatcacttccaaaataaatgatgaattccctactcctagagattgcatcaccctcttccctcttcagcatcagtcatttcagagccagccctagtgactttgtaattatggttcccagaatataaacccttatgaaggattttttgacttttccttgatgcttccatgatgtcagtaacatttcagtggttccatgacccatcttctcctgctcagagaccacagtggacttcttttttcttctgctggcctttgtttatctcctttaatcataaaggaatcttcagcaggagtgtttctccctttcccttcttgctctcctttctctactgttgtattttcttgctactactttatttgaccattggtcatttcatatttcttccactcttcatctccaagattatgcttatctattgttgaaagaaaacagagctgtgtcctattcattctctgattcacctttttccttttcattatggtttctcagttctgttctgtgtattaatctattgtttcattgacaaattgcccaaaagttagcagcttaaaataaaacaaaaacatttattatgtcagtttctgttatctcacagacatggcttaactcagtgcctctggctctgcttctcttgtcaggtaccagccaagttgtgggctggggttggaggcttagctggggagagtttaccttgcagctcactggtgtggatgccggcacgtctcaatctctcactatttgagcctctccacagggttgcctcacagcgttgcagttgcctttccccaggccgagtgatccaagagggaaccagcaaaagcacccaagacagaaaccacaatctttttatagtttattctcagagttgacacctcgtcacttctgccatattaagcgagttagtaaatccagtccacattcatggggaagagattacaaaggaatatgagtaccgggagatcgagatcatgaggagctatcctggaatctggctaccacactcttcctctggccccccagtgacttatatcccttcaatgtgcagaatatactcacccctccaaggattgcaaagtctcatcccattgcagtgtgagctcaatatccaaaatcttgtcatctaaatcaggtccaggtgcagttggggctcctcagttttaattccttaagtacagctctttgagtacatttcttcttcttaacctgtgaaaccttaatttatttaaagcgctcctatgtgactgaatcgtattctgaggcaccatctttgtttcttctgaggtcttcacgaatggttttaagtcacacccttgatttcatctttaatcttccttctctcaattcaacgccttcaatttgatcttgctcaaagattctccagtcttaagtcatctgcgctttctgactttctcaaattctctcagcccaaccgctgcatagtaacctacggtagatcttccagcatctctctttctgtagaatattaccaagatactctgaagaatacatgcatggcagaaagtactttggggttcatgccactaattgacactttatcatgaaaagattaaaatgttctcatttgtatttct

SEQ ID NO: 16141 - RNA, 3990 nt, Homo sapiens
  source 1..3990: mol_type = other RNA
gctgggattacaggcatgagccgcagtgcctggcttatgtgtgatcttttaaaggactgtctattaccaatccaaagttactatatttttcattgcaacaatttggggtcttattcttattgtaggtgctttaaactcattacaccagagtgttattctacccaaagtttgtgacccagctcaggataactgtgagaagcaatttagtgtagtgttgcttaacttgcccaccgaagtggacaagttaaatttccctgtgactcagtcaccttcttggtaaatgataacaattatttcttcctcacagagttgtaatgatgattaaataagactgtgcttgataagcacttcaaacagtggttatcagagagtaatcactgaagtgttaattattatatagttaataattatattataatcttttttattttgtccattattttttcttcctgggaagggacatgcagaaaggtatacatgtttaatatataatcatcttggttttttttctccaaccattaaatattttgctcaaaggccctatactagttttagtttcaatcattcttctggaaacctacagggtaacacatccgtagctcttcaatttatttcctcaaggtggggtttaatttttccctagcttatcccactaatcataccatagtcatgccctctctgacttttgcctctaatcaatgtctacctacaggacttacttgcacgtagtcttcttcatactccattggctttcgtttttttcttgctttccccttgattttcttcttgtttgttccttgctctttctggactcattggtaaaacaataaagaccttttattgagcagttaatactgttactgtataaggcacactgtaacataatcctcacggcatccctaggaggtaggtggtacccactttacaaagaaccagaggctcagagagatgggttctgggggtcatggcccatctgcttggctgtgagccagactccaaggatactgttgctttcactttcctttttacctgtcctctctctttcagctcaggaaaattggattaaccgtgttctcatgtgttttgttggtcacatgccattgctattttttgtcaggcatactgtctgtcctttcaggagtccttctctaattgtttacacgcatagaacttgagtctccagctggttcgtaagtcccttggggccagggtttcttttgtgtccactatagtacctaacacagtttggggctcttatttggcagatatgaccagatgtatgttttctaaatataactgcattttttctggatcaattttttaaaaatgttatgctatatttaaattttagatttgtttcaactttgcttaagactgtactattccttcagtttttctttatgcttgtacaggaactacttggcatgatgctgtcagctgtaatatacatttaggctttaatatcaccaggcaagagcatctgtcaagatagatgatgttccctcctttgccatagctgggcctcacatttctgtcgctgaatacatgcctctagtttgttcagtattttaagcagcagatttataactttaaagtttttaaatccatgcaactacctcatctctagcaaccatttcacatctaaataatcatccttggcctgcttaataatgtgagtataaagatttgccaatagttctttttcccccagtaatcacttccaaaataaatgatgaattccctactcctagagattgcatcaccctcttccctcttcagcatcagtcatttcagagccagccctagtgactttgtaattatggttcccagaatataaacccttatgaaggattttttgacttttccttgatgcttccatgatgtcagtaacatttcagtggttccatgacccatcttctcctgctcagagaccacagtggacttcttttttcttctgctggcctttgtttatctcctttaatcataaaggaatcttcagcaggagtgtttctccctttcccttcttgctctcctttctctactgttgtattttcttgctactactttatttgaccattggtcatttcatatttcttccactcttcatctccaagattatgcttatctattgttgaaagaaaacagagctgtgtcctattcattctctgattcacctttttccttttcattatggtttctcagttctgttctgtgtattaatctattgtttcattgacaaattgcccaaaagttagcagcttaaaataaaacaaaaacatttattatgtcagtttctgttatctcacagacatggcttaactcagtgcctctggctctgcttctcttgtcaggtaccagccaagttgtgggctggggttggaggcttagctggggagagtttaccttgcagctcactggtgtggatgccggcacgtctcaatctctcactatttgagcctctccacagggttgcctcacagcgttgcagttgcctttccccaggccgagtgatccaagagggaaccagcaaaagcacccaagacagaaaccacaatctttttatagtttattctcagagttgacacctcgtcacttctgccatattaagcgagttagtaaatccagtccacattcatggggaagagattacaaaggaatatgagtaccgggagatcgagatcatgaggagctatcctggaatctggctaccacactcttcctctggccccccagtgacttatatcccttcaatgtgcagaatatactcacccctccaaggattgcaaagtctcatcccattgcagtgtgagctcaatatccaaaatcttgtcatctaaatcaggtccaggtgcagttggggctcctcagttttaattccttaagtacagctctttgagtacatttcttcttcttaacctgtgaaaccttaatttatttaaagcgctcctatgtgactgaatcgtattctgaggcaccatctttgtttcttctgaggtcttcacgaatggttttaagtcacacccttgatttcatctttaatcttccttctctcaattcaacgccttcctgtaagacccaagaagaaatcaggtgtcaccttcaacactatttgaaaatctccttagctagattacccttgccaatagacacattttccatataatttcagaaaactgtattgctaaactttctaccactgcataacaaagagcccctttcctttagtttccaataagatttttctttcttcaagccctcaccttccatgtcttcaaagtccaaaatttcatagtgttgttcaagcgcattcttcatcaatcactttacttttgacacatttcagagtagtttgcaaaatcagtacactcactccagatacttcagcatgcatatcactgactaatgtttaatatttatcttaaagtatgtatattttcttttgaggtaaagttaatatacaataaatgtacaaatgtcaaatataccattcaatgaattttgacaaataaatacaactatgtaattcaaagcccagtctggattgaaaaaacaggatcatcacccccagaatcctttcatgccacctgggtcaatcacgatgctaaattccttgcctcagaggcaacaactgttccgatattttttctaaaaaattaattttgcctattctaaaatggcatataaatggaatcatacagttacatgctgttttgtttaaggcttctttcattcgacacagtattatttagattcctccatgtcagtgtatagtatttcacttctttttatcgctgagcacattaagtctgctagggctgccataacaaaatgccatagacagggtggctgaaacaacagttctaaaagctagaagtctgcgatcaagatgtctacaggtgtggtttctcctgaggcctctccccttcacttgcagatggccttctcactatgtcttcacatggtcttttctctgtctgtgcatatccctgg

SEQ ID NO: 16142 - RNA, 3767 nt, Homo sapiens
  source 1..3767: mol_type = other RNA
gctgggattacaggcatgagccgcagtgcctggcttatgtgtgatcttttaaaggactgtctattaccaatccaaagttactatatttttcattgcaacaatttggggtcttattcttattgtaggtgctttaaactcattacaccagagtgttattctacccaaagtttgtgacccagctcaggataactgtgagaagcaatttagtgtagtgttgcttaacttgcccaccgaagtggacaagttaaatttccctgtgactcagtcaccttcttggtaaatgataacaattatttcttcctcacagagttgtaatgatgattaaataagactgtgcttgataagcacttcaaacagtggttatcagagagtaatcactgaagtgttaattattatatagttaataattatattataatcttttttattttgtccattattttttcttcctgggaagggacatgcagaaaggtatacatgtttaatatataatcatcttggttttttttctccaaccattaaatattttgctcaaaggccctatactagttttagtttcaatcattcttctggaaacctacagggtaacacatccgtagctcttcaatttatttcctcaaggtggggtttaatttttccctagcttatcccactaatcataccatagtcatgccctctctgacttttgcctctaatcaatgtctacctacaggacttacttgcacgtagtcttcttcatactccattggctttcgtttttttcttgctttccccttgattttcttcttgtttgttccttgctctttctgtcctctctctttcagctcaggaaaattggattaaccgtgttctcatgtgttttgttggtcacatgccattgctattttttgtcaggcatactgtctgtcctttcaggagtccttctctaattgtttacacgcatagaacttgagtctccagctggttcgtaagtcccttggggccagggtttcttttgtgtccactatagtacctaacacagtttggggctcttatttggcagatatgaccagatgtatgttttctaaatataactgcattttttctggatcaattttttaaaaatgttatgctatatttaaattttagatttgtttcaactttgcttaagactgtactattccttcagtttttctttatgcttgtacaggaactacttggcatgatgctgtcagctgtaatatacatttaggctttaatatcaccaggcaagagcatctgtcaagatagatgatgttccctcctttgccatagctgggcctcacatttctgtcgctgaatacatgcctctagtttgttcagtattttaagcagcagatttataactttaaagtttttaaatccatgcaactacctcatctctagcaaccatttcacatctaaataatcatccttggcctgcttaataatgtgagtataaagatttgccaatagttctttttcccccagtaatcacttccaaaataaatgatgaattccctactcctagagattgcatcaccctcttccctcttcagcatcagtcatttcagagccagccctagtgactttgtaattatggttcccagaatataaacccttatgaaggattttttgacttttccttgatgcttccatgatgtcagtaacatttcagtggttccatgacccatcttctcctgctcagagaccacagtggacttcttttttcttctgctggcctttgtttatctcctttaatcataaaggaatcttcagcaggagtgtttctccctttcccttcttgctctcctttctctactgttgtattttcttgctactactttatttgaccattggtcatttcatatttcttccactcttcatctccaagattatgcttatctattgttgaaagaaaacagagctgtgtcctattcattctctgattcacctttttccttttcattatggtttctcagttctgttctgtgtattaatctattgtttcattgacaaattgcccaaaagttagcagcttaaaataaaacaaaaacatttattatgtcagtttctgttatctcacagacatggcttaactcagtgcctctggctctgcttctcttgtcaggtaccagccaagttgtgggctggggttggaggcttagctggggagagtttaccttgcagctcactggtgtggatgccggcacgtctcaatctctcactatttgagcctctccacagggttgcctcacagcgttgcagttgcctttccccaggccgagtgatccaagagggaaccagcaaaagcacccaagacagaaaccacaatctttttatagtttattctcagagttgacacctcgtcacttctgccatattaagcgagttagtaaatccagtccacattcatggggaagagattacaaaggaatatgagtaccgggagatcgagatcatgaggagctatcctggaatctggctaccacactcttcctctggccccccagtgacttatatcccttcaatgtgcagaatatactcacccctccaaggattgcaaagtctcatcccattgcagtgtgagctcaatatccaaaatcttgtcatctaaatcaggtccaggtgcagttggggctcctcagttttaattccttaagtacagctctttgagtacatttcttcttcttaacctgtgaaaccttaatttatttaaagcgctcctatgtgactgaatcgtattctgaggcaccatctttgtttcttctgaggtcttcacgaatggttttaagtcacacccttgatttcatctttaatcttccttctctcaattcaacgccttcctgtaagacccaagaagaaatcaggtgtcaccttcaacactatttgaaaatctccttagctagattacccttgccaatagacacattttccatataatttcagaaaactgtattgctaaactttctaccactgcataacaaagagcccctttcctttagtttccaataagatttttctttcttcaagccctcaccttccatgtcttcaaagtccaaaatttcatagtgttgttcaagcgcattcttcatcaatcactttacttttgacacatttcagagtagtttgcaaaatcagtacactcactccagatacttcagcatgcatatcactgactaatgtttaatatttatcttaaagtatgtatattttcttttgaggtaaagttaatatacaataaatgtacaaatgtcaaatataccattcaatgaattttgacaaataaatacaactatgtaattcaaagcccagtctggattgaaaaaacaggatcatcacccccagaatcctttcatgccacctgggtcaatcacgatgctaaattccttgcctcagaggcaacaactgttccgatattttttctaaaaaattaattttgcctattctaaaatggcatataaatggaatcatacagttacatgctgttttgtttaaggcttctttcattcgacacagtattatttagattcctccatgtcagtgtatagtatttcacttctttttatcgctgagcacattaagtctgctagggctgccataacaaaatgccatagacagggtggctgaaacaacagttctaaaagctagaagtctgcgatcaagatgtctacaggtgtggtttctcctgaggcctctccccttcacttgcagatggccttctcactatgtcttcacatggtcttttctctgtctgtgcatatccctgg

SEQ ID NO: 16143 - RNA, 4622 nt, Homo sapiens
  source 1..4622: mol_type = other RNA
gctgggattacaggcatgagccgccacacccagcagaattttaatttaaaagctcagcttaaacacctcatgatgcttacacatttggtacatttttaacaatcgttgattgttcaactccatccgtctcagagttaaagacacaggataaggaaaacatctccttatccaagtgatttggggtggtattcccagctgtctgaggctgtacattgaccaattattttggccatgactcagagttcccctatcctgctatcctgagatcatgagaggccatcacagagtccacttttatcatctctatgccaataagggctctaaatggggtggtgtgacagcccatgtgccctacgttcaagttacctaatttttccaaagaactgagttttgctgataccctccactcccacccagctttcctcaccatttcattggattctgcttgtctaaatattgctgattttgttctgatttttctcttttttttttttttttgagacagagtctcactctgtcacctaggctggagtgcagtggcgcaatctccactcactgcaagctccgcctcccgagttccagttattctgcatcagcctcccgggtagccaggactacaggcacgtgcaagcacgcccggctaattttgtatttttagtagagacaggtttcaccatgttggtcaggctggtcttgaactcctgacctcgtgatccgcccaccctggcctcccaaagtgctgggattacaggcgtgagccaccgtgcccagcctttttttttttcttttctgagacagagtctcactctctcgtccagactggagtgcaggggcacaatctcagctaatggcaatctccacctcctgggcttcagcgattcttgtgcctcagcctcccaagtagctaggattacagaagtgcgtcaccatagctggctaatttttgtatttttagtagagacagggtttcactatgttggccaggctggtcttgaactcctgatctcaggtgggccaggtatggtggctcacgcctgtaatcccagcactttgggaggctgaagcgggcagatcacctgaggtcaggactttgagaccagcatgtccaacatggtgaaaccccgtctctactaaaaatacaaaagttagctgggcgtggtggtgaacgcctataatcccagctacttgggtggctgaggcaggagaatcacttgaccctgggaggcggaggttgcagtgagccaagattgtgccattgcactccagcctgggtgacagagcaagactccatctcaaaaaaaaataataaaattagctggaaaaaaatatttagccaggcatcgtggtgcacgcctgtagtcccagctattctggagggtgaggtgggaagatggttgagcctgggaggatgacggtgcagtgagtcatgtttgcaccattgcactccagcctgggtgacagagcaagactctgtctaaaaaaaacaggccggaaacagtggctcatgcctatattcccagtactttggaaggccgaggtaggcggatcacctcaggtcaggagttccagaccagcctggccaacatagtgaaaccctgtctctactaaaaatacaaaaattagccaggcttggtggtgcacaccggtaatcccagcaactctggagactaaggcaggaagaatcgcttgacccaggagggtcgaggctgcaatgagttgaaaccgcgccactgcactctagcctgggcgacagtgcgaggccctgtctcaaaaataaaataaaataaataaattagccagatactgtgtgcacgcctgcagtcccagctattctggaagctgaggtgggaagatggttaagcctgagaggacaaagctgcagtgagtcatgtttgcatcactgcactccagcctgggtgacagagcaagaccctgtctaaaaaacaaaaacaggccgggtgtggtggctcatgcctgccatcccagtgctttgggaggcagaggttggcataatcccagcgctctgggaggctgaggtgggcggatcacctgaggtcaggagttccagaccagcctggccaacatggtgaaaccctgtctctactaaaaatacaaaaattagccaggcatggtggtacacatctgtaatcccagctacttgagaagctgaggcaggagaatcgcttgaacctgggaggcagaggttgcagtgagctgagattgtgccactgcactccaacctggatgacggagtgagactccgtctcagaaaaaaaaaaaaccaaaacaggccgggtgtggtggctcacggctgtaatcccagtactttgggaggccaagccaggcggatcacgaggtcaggagattgagaccatcctggctaacacggtgcaacaccgtctctactaaaaatacaaaaaaattagctgggcgtggtggtgggcacctgtagtcccagctactcgggaggctgaggcaggagaatggcgtgaacctgggaagcggaggttgcagtgagcctagatcgcaccactgcactccagcctgggccacaaagcaagtctcaaaaacaaaaacaaaaacaaaaaaatgattaacatttcaatcagtcaatgggtagactttgagtcacgctgattatccaccacaattgtgggcggagctcattcaataaactgaagacctttaagagaaaagactgaggtcccggccaggtgcggtggctcacgcctgtaatcccagcactttgggaggctgagccaggccaacatggtgaaacctcatctcggatacaaaaaattagccaggtgtggtggcgggcgcctgtgaccccagctacttgggaggctgaggcaggagaatcacttgaacctgggaggcggaggctgcagtgagcaaagatggcgccactgcactccagcctgggcaacaacagaaaaacaacaaaaatcatctcattttcatctgtgtcttccagtattaaagaggttgagtgtcatttctggcttactagccatttggatttcttctgatacacacttcatctcatttgcctaattttgtcgttgtcttcttattgctttctaagggctctctgtatactatggatattagtccttggttaatgacactgcaaatacttacaattttttttaatttttaattttcgtgggcacatagtttattgagaatttttttttttttgagatggcaggggtctcatatgttccccagactagagtgcagtggctattcacaggcgccgtctagcgcactacaaccttaaactcctgggctcaagcaattctcctgcctcagccttgggagtagctgggattacaagtgcccgccaccacgcctggtctgccaatactttctatcagtctgtcatgtttactgtcttttcctccatacagaagtttttccttctcagttgggtcaagtccattgacctttctgttacagcttgagttttgtgtcttacgtagaaaaggtgcccctgctctcactttctgcacagctatcaggtccagctcatagcagttcttctatttatccatccactgccccaggagctgcctgggcattcactgccccgcacccctctccagccccaaggtagagctcgggccctgggagtcccaggaccatcccggactggggagctgcttggtgtccagccccgggctcaagctcttctccagctctgcagctacctgaggggtagcagcccggatagcatcctggatgttggttaggtcccactgggtcctcaggagggcactgtctagcgtgaagaagccgtcgcgcgtgcgccgcacttgggtgcagacagcagtggtctttagttccaggccgatttcatgaaccaacttccgcagctctttctgcgtctcatgcatgcactgcacctctaagaggaattccggaggtgcaaagtagaggcatcggatgccagttatcagcatcggggacttgttcatgggccggatcaggcctctcacggccatctcataggcctcctgggtcttcaggtcgaggttggagtacatcaccagggccttctgatgggagccttggataacggccagaatgcggtccagcttctctctggtcacgtggtcataggttgtcttctctaccagcctcccgtcctcacggaagtcatctgtagctttgcccaggaggccacgcactgtgtaatccttggtaagatgagcattgtacatatcggtgaggagcctgcatccatgtcccacgccgagcacaagtactccagaagcctgggcatccaaccgatgtcccacgccaaccttgagatgggcgaatgctggtccacataccagtggatggttgatgaaagagggtacgctggtggctgtgagggtcagctccttctcttcgctgccttccatggggcccagcaagaagcgaacacgctgtttaggagcgggaggcttcctggcattgagacccttcagaagttgtagctccactgtatcccgcaggtgcttccattttagccccgggggcttatagaccgcgaaaagcccatgcagccgcgacaagccagcagaccccatacttgaagatcacagcacccgctggacctggacggaagt

SEQ ID NO: 16144 - RNA, 4837 nt, Homo sapiens
  source 1..4837: mol_type = other RNA
gctgggattacaggcatgagccgccacacccagcagaattttaatttaaaagctcagcttaaacacctcatgatgcttacacatttggtacatttttaacaatcgttgattgttcaactccatccgtctcagagttaaagacacaggataaggaaaacatctccttatccaagtgatttggggtggtattcccagctgtctgaggctgtacattgaccaattattttggccatgactcagagttcccctatcctgctatcctgagatcatgagaggccatcacagagtccacttttatcatctctatgccaataagggctctaaatggggtggtgtgacagcccatgtgccctacgttcaagttacctaatttttccaaagaactgagttttgctgataccctccactcccacccagctttcctcaccatttcattggattctgcttgtctaaatattgctgattttgttctgatttttctcttttttttttttttttgagacagagtctcactctgtcacctaggctggagtgcagtggcgcaatctccactcactgcaagctccgcctcccgagttccagttattctgcatcagcctcccgggtagccaggactacaggcacgtgcaagcacgcccggctaattttgtatttttagtagagacaggtttcaccatgttggtcaggctggtcttgaactcctgacctcgtgatccgcccaccctggcctcccaaagtgctgggattacaggcgtgagccaccgtgcccagcctttttttttttcttttctgagacagagtctcactctctcgtccagactggagtgcaggggcacaatctcagctaatggcaatctccacctcctgggcttcagcgattcttgtgcctcagcctcccaagtagctaggattacagaagtgcgtcaccatagctggctaatttttgtatttttagtagagacagggtttcactatgttggccaggctggtcttgaactcctgatctcaggtgggccaggtatggtggctcacgcctgtaatcccagcactttgggaggctgaagcgggcagatcacctgaggtcaggactttgagaccagcatgtccaacatggtgaaaccccgtctctactaaaaatacaaaagttagctgggcgtggtggtgaacgcctataatcccagctacttgggtggctgaggcaggagaatcacttgaccctgggaggcggaggttgcagtgagccaagattgtgccattgcactccagcctgggtgacagagcaagactccatctcaaaaaaaaataataaaattagctggaaaaaaatatttagccaggcatcgtggtgcacgcctgtagtcccagctattctggagggtgaggtgggaagatggttgagcctgggaggatgacggtgcagtgagtcatgtttgcaccattgcactccagcctgggtgacagagcaagactctgtctaaaaaaaacaggccggaaacagtggctcatgcctatattcccagtactttggaaggccgaggtaggcggatcacctcaggtcaggagttccagaccagcctggccaacatagtgaaaccctgtctctactaaaaatacaaaaattagccaggcttggtggtgcacaccggtaatcccagcaactctggagactaaggcaggaagaatcgcttgacccaggagggtcgaggctgcaatgagttgaaaccgcgccactgcactctagcctgggcgacagtgcgaggccctgtctcaaaaataaaataaaataaataaattagccagatactgtgtgcacgcctgcagtcccagctattctggaagctgaggtgggaagatggttaagcctgagaggacaaagctgcagtgagtcatgtttgcatcactgcactccagcctgggtgacagagcaagaccctgtctaaaaaacaaaaacaggccgggtgtggtggctcatgcctgccatcccagtgctttgggaggcagaggttggcataatcccagcgctctgggaggctgaggtgggcggatcacctgaggtcaggagttccagaccagcctggccaacatggtgaaaccctgtctctactaaaaatacaaaaattagccaggcatggtggtacacatctgtaatcccagctacttgagaagctgaggcaggagaatcgcttgaacctgggaggcagaggttgcagtgagctgagattgtgccactgcactccaacctggatgacggagtgagactccgtctcagaaaaaaaaaaaaccaaaacaggccgggtgtggtggctcacggctgtaatcccagtactttgggaggccaagccaggcggatcacgaggtcaggagattgagaccatcctggctaacacggtgcaacaccgtctctactaaaaatacaaaaaaattagctgggcgtggtggtgggcacctgtagtcccagctactcgggaggctgaggcaggagaatggcgtgaacctgggaagcggaggttgcagtgagcctagatcgcaccactgcactccagcctgggccacaaagcaagtctcaaaaacaaaaacaaaaacaaaaaaatgattaacatttcaatcagtcaatgggtagactttgagtcacgctgattatccaccacaattgtgggcggagctcattcaataaactgaagacctttaagagaaaagactgaggtcccggccaggtgcggtggctcacgcctgtaatcccagcactttgggaggctgagccaggccaacatggtgaaacctcatctcggatacaaaaaattagccaggtgtggtggcgggcgcctgtgaccccagctacttgggaggctgaggcaggagaatcacttgaacctgggaggcggaggctgcagtgagcaaagatggcgccactgcactccagcctgggcaacaacagaaaaacaacaaaaatcatctcattttcatctgtgtcttccagtattaaagaggttgagtgtcatttctggcttactagccatttggatttcttctgatacacacttcatctcatttgcctaattttgtcgttgtcttcttattgctttctaagggctctctgtatactatggatattagtccttggttaatgacactgcaaatacttacaattttttttaatttttaattttcgtgggcacatagtttattgagaatttttttttttttgagatggcaggggtctcatatgttccccagactagagtgcagtggctattcacaggcgccgtctagcgcactacaaccttaaactcctgggctcaagcaattctcctgcctcagccttgggagtagctgggattacaagtgcccgccaccacgcctggtctgccaatactttctatcagtctgtcatgtttactgtcttttcctccatacagaagtttttccttctcagttgggtcaagtccattgacctttctgttacagcttgagttttgtgtcttacgtagaaaaggtgcccctgctctcactttctgcacagctatcaggtccagctcatagcagttcttctatttatccatccactgccccaggagctgcctgggcattcactgccccgcacccctctccagccccaaggtagagctcgggccctgggagtcccaggaccatcccggactggggagctgcttggtgtccagccccgggctcaagctcttctccagctctgcagctacctgaggggtagcagcccggatagcatcctggatgttggttaggtcccactgggtcctcaggagggcactgtctagcgtgaagaagccgtcgcgcgtgcgccgcacttgggtgcagacagcagtggtctttagttccaggccgatttcatgaaccaacttccgcagctctttctgcgtctcatgcatgcactgcacctctaagaggaattccggaggtgcaaagtagaggcatcggatgccagttatcagcatcggggacttgttcatgggccggatcaggcctctcacggccatctcataggcctcctgggtcttcaggtcgaggttggagtacatcaccagggccttctgatgggagccttggataacggccagaatgcggtccagcttctctctggtcacgtggtcataggttgtcttctctaccagcctcccgtcctcacggaagtcatctgtagctttgcccaggaggccacgcactgtgtaatccttggtaagatgagcattgtacatatcggtgaggagcctgcatccatgtcccacgccgagcacaagtactccagaagcctgggcatccaaccgatgtcccacgccaaccttgagatgggcgaatgctggtccacataccagtggatggttgatgaaagagggtacgctggtggctgtgagggtcagctccttctcttcgctgccttccatggggcccagcaagaagcgaacacgctgtttaggagcgggaggcttcctggcattgagactgtaacgtcaaactcttgggctcaagcgatcctcctgcctcagcctccagagtagctgggattacaggcgtgcaccacgatgctgaccaggaatatcttgttctgtccaaacacttgggggattagacaacagggaagtatgatgtagaagacaaagcagaagcccatggtgcagagggcagtatagcagtagttaagaaacaggcggattcaaacagactctacaacgtagtaaccgtgtgacaaggaacaatactgagtcagtttccccctcggaaaacagaggaaagtgaggagtaagaaagcacagagaacaggcgtttgggaaagcgctctgcccaggtgaataggtcacgtgatttt

SEQ ID NO: 16145 - RNA, 4490 nt, Homo sapiens
  source 1..4490: mol_type = other RNA
gctgggattacaggcatgagccgccacacccagcagaattttaatttaaaagctcagcttaaacacctcatgatgcttacacatttggtacatttttaacaatcgttgattgttcaactccatccgtctcagagttaaagacacaggataaggaaaacatctccttatccaagtgatttggggtggtattcccagctgtctgaggctgtacattgaccaattattttggccatgactcagagttcccctatcctgctatcctgagatcatgagaggccatcacagagtccacttttatcatctctatgccaataagggctctaaatggggtggtgtgacagcccatgtgccctacgttcaagttacctaatttttccaaagaactgagttttgctgataccctccactcccacccagctttcctcaccatttcattggattctgcttgtctaaatattgctgattttgttctgatttttctcttttttttttttttttgagacagagtctcactctgtcacctaggctggagtgcagtggcgcaatctccactcactgcaagctccgcctcccgagttccagttattctgcatcagcctcccgggtagccaggactacaggcacgtgcaagcacgcccggctaattttgtatttttagtagagacaggtttcaccatgttggtcaggctggtcttgaactcctgacctcgtgatccgcccaccctggcctcccaaagtgctgggattacaggcgtgagccaccgtgcccagcctttttttttttcttttctgagacagagtctcactctctcgtccagactggagtgcaggggcacaatctcagctaatggcaatctccacctcctgggcttcagcgattcttgtgcctcagcctcccaagtagctaggattacagaagtgcgtcaccatagctggctaatttttgtatttttagtagagacagggtttcactatgttggccaggctggtcttgaactcctgatctcaggtgggccaggtatggtggctcacgcctgtaatcccagcactttgggaggctgaagcgggcagatcacctgaggtcaggactttgagaccagcatgtccaacatggtgaaaccccgtctctactaaaaatacaaaagttagctgggcgtggtggtgaacgcctataatcccagctacttgggtggctgaggcaggagaatcacttgaccctgggaggcggaggttgcagtgagccaagattgtgccattgcactccagcctgggtgacagagcaagactccatctcaaaaaaaaataataaaattagctggaaaaaaatatttagccaggcatcgtggtgcacgcctgtagtcccagctattctggagggtgaggtgggaagatggttgagcctgggaggatgacggtgcagtgagtcatgtttgcaccattgcactccagcctgggtgacagagcaagactctgtctaaaaaaaacaggccggaaacagtggctcatgcctatattcccagtactttggaaggccgaggtaggcggatcacctcaggtcaggagttccagaccagcctggccaacatagtgaaaccctgtctctactaaaaatacaaaaattagccaggcttggtggtgcacaccggtaatcccagcaactctggagactaaggcaggaagaatcgcttgacccaggagggtcgaggctgcaatgagttgaaaccgcgccactgcactctagcctgggcgacagtgcgaggccctgtctcaaaaataaaataaaataaataaattagccagatactgtgtgcacgcctgcagtcccagctattctggaagctgaggtgggaagatggttaagcctgagaggacaaagctgcagtgagtcatgtttgcatcactgcactccagcctgggtgacagagcaagaccctgtctaaaaaacaaaaacaggccgggtgtggtggctcatgcctgccatcccagtgctttgggaggcagaggttggcataatcccagcgctctgggaggctgaggtgggcggatcacctgaggtcaggagttccagaccagcctggccaacatggtgaaaccctgtctctactaaaaatacaaaaattagccaggcatggtggtacacatctgtaatcccagctacttgagaagctgaggcaggagaatcgcttgaacctgggaggcagaggttgcagtgagctgagattgtgccactgcactccaacctggatgacggagtgagactccgtctcagaaaaaaaaaaaaccaaaacaggccgggtgtggtggctcacggctgtaatcccagtactttgggaggccaagccaggcggatcacgaggtcaggagattgagaccatcctggctaacacggtgcaacaccgtctctactaaaaatacaaaaaaattagctgggcgtggtggtgggcacctgtagtcccagctactcgggaggctgaggcaggagaatggcgtgaacctgggaagcggaggttgcagtgagcctagatcgcaccactgcactccagcctgggccacaaagcaagtctcaaaaacaaaaacaaaaacaaaaaaatgattaacatttcaatcagtcaatgggtagactttgagtcacgctgattatccaccacaattgtgggcggagctcattcaataaactgaagacctttaagagaaaagactgaggtcccggccaggtgcggtggctcacgcctgtaatcccagcactttgggaggctgagccaggccaacatggtgaaacctcatctcggatacaaaaaattagccaggtgtggtggcgggcgcctgtgaccccagctacttgggaggctgaggcaggagaatcacttgaacctgggaggcggaggctgcagtgagcaaagatggcgccactgcactccagcctgggcaacaacagaaaaacaacaaaaatcatctcattttcatctgtgtcttccagtattaaagaggttgagtgtcatttctggcttactagccatttggatttcttctgatacacacttcatctcatttgcctaattttgtcgttgtcttcttattgctttctaagggctctctgtatactatggatattagtccttggttaatgacactgcaaatacttacaattttttttaatttttaattttcgtgggcacatagtttattgagaatttttttttttttgagatggcaggggtctcatatgttccccagactagagtgcagtggctattcacaggcgccgtctagcgcactacaaccttaaactcctgggctcaagcaattctcctgcctcagccttgggagtagctgggattacaagtgcccgccaccacgcctggtctgccaatactttctatcagtctgtcatgtttactgtcttttcctccatacagaagtttttccttctcagttgggtcaagtccattgacctttctgttacagcttgagttttgtgtcttacgtagaaaaggtgcccctgctctcactttctgcacagctatcaggtccagctcatagcagttcttctatttatccatccactgccccaggagctgcctgggcattcactgccccgcacccctctccagccccaaggtagagctcgggccctgggagtcccaggaccatcccggactggggagctgcttggtgtccagccccgggctcaagctcttctccagctctgcagctacctgaggggtagcagcccggatagcatcctggatgttggttaggtcccactgggtcctcaggagggcactgtctagcgtgaagaagccgtcgcgcgtgcgccgcacttgggtgcagacagcagtggtctttagttccaggccgatttcatgaaccaacttccgcagctctttctgcgtctcatgcatgcactgcacctctaagaggaattccggaggtgcaaagtagaggcatcggatgccagttatcagcatcggggacttgttcatgggccggatcaggcctctcacggccatctcataggcctcctgggtcttcaggtcgaggttggagtacatcaccagggccttctgatgggagccttggataacggccagaatgcggtccagcttctctctggtcacgtggtcataggttgtcttctctaccagcctcccgtcctcacggaagtcatctgtagctttgcccaggaggccacgcactgtgtaatccttggtaagatgagcattgtacatatcggtgaggagcctgcatccatgtcccacgccgagcacaagtactccagaagcctgggcatccaaccgatgtcccacgccaaccttgagatgggcgaatgctggtccacataccttcagaagttgtagctccactgtatcccgcaggtgcttccattttagccccgggggcttatagaccgcgaaaagcccatgcagccgcgacaagccagcagaccccatacttgaagatcacagcacccgctggacctggacggaagt

SEQ ID NO: 16146 - RNA, 4697 nt, Homo sapiens
  source 1..4697: mol_type = other RNA
gctgggattacaggcatgagccgccacacccagcagaattttaatttaaaagctcagcttaaacacctcatgatgcttacacatttggtacatttttaacaatcgttgattgttcaactccatccgtctcagagttaaagacacaggataaggaaaacatctccttatccaagtgatttggggtggtattcccagctgtctgaggctgtacattgaccaattattttggccatgactcagagttcccctatcctgctatcctgagatcatgagaggccatcacagagtccacttttatcatctctatgccaataagggctctaaatggggtggtgtgacagcccatgtgccctacgttcaagttacctaatttttccaaagaactgagttttgctgataccctccactcccacccagctttcctcaccatttcattggattctgcttgtctaaatattgctgattttgttctgatttttctcttttttttttttttttgagacagagtctcactctgtcacctaggctggagtgcagtggcgcaatctccactcactgcaagctccgcctcccgagttccagttattctgcatcagcctcccgggtagccaggactacaggcacgtgcaagcacgcccggctaattttgtatttttagtagagacaggtttcaccatgttggtcaggctggtcttgaactcctgacctcgtgatccgcccaccctggcctcccaaagtgctgggattacaggcgtgagccaccgtgcccagcctttttttttttcttttctgagacagagtctcactctctcgtccagactggagtgcaggggcacaatctcagctaatggcaatctccacctcctgggcttcagcgattcttgtgcctcagcctcccaagtagctaggattacagaagtgcgtcaccatagctggctaatttttgtatttttagtagagacagggtttcactatgttggccaggctggtcttgaactcctgatctcaggtgggccaggtatggtggctcacgcctgtaatcccagcactttgggaggctgaagcgggcagatcacctgaggtcaggactttgagaccagcatgtccaacatggtgaaaccccgtctctactaaaaatacaaaagttagctgggcgtggtggtgaacgcctataatcccagctacttgggtggctgaggcaggagaatcacttgaccctgggaggcggaggttgcagtgagccaagattgtgccattgcactccagcctgggtgacagagcaagactccatctcaaaaaaaaataataaaattagctggaaaaaaatatttagccaggcatcgtggtgcacgcctgtagtcccagctattctggagggtgaggtgggaagatggttgagcctgggaggatgacggtgcagtgagtcatgtttgcaccattgcactccagcctgggtgacagagcaagactctgtctaaaaaaaacaggccggaaacagtggctcatgcctatattcccagtactttggaaggccgaggtaggcggatcacctcaggtcaggagttccagaccagcctggccaacatagtgaaaccctgtctctactaaaaatacaaaaattagccaggcttggtggtgcacaccggtaatcccagcaactctggagactaaggcaggaagaatcgcttgacccaggagggtcgaggctgcaatgagttgaaaccgcgccactgcactctagcctgggcgacagtgcgaggccctgtctcaaaaataaaataaaataaataaattagccagatactgtgtgcacgcctgcagtcccagctattctggaagctgaggtgggaagatggttaagcctgagaggacaaagctgcagtgagtcatgtttgcatcactgcactccagcctgggtgacagagcaagaccctgtctaaaaaacaaaaacaggccgggtgtggtggctcatgcctgccatcccagtgctttgggaggcagaggttggcataatcccagcgctctgggaggctgaggtgggcggatcacctgaggtcaggagttccagaccagcctggccaacatggtgaaaccctgtctctactaaaaatacaaaaattagccaggcatggtggtacacatctgtaatcccagctacttgagaagctgaggcaggagaatcgcttgaacctgggaggcagaggttgcagtgagctgagattgtgccactgcactccaacctggatgacggagtgagactccgtctcagaaaaaaaaaaaaccaaaacaggccgggtgtggtggctcacggctgtaatcccagtactttgggaggccaagccaggcggatcacgaggtcaggagattgagaccatcctggctaacacggtgcaacaccgtctctactaaaaatacaaaaaaattagctgggcgtggtggtgggcacctgtagtcccagctactcgggaggctgaggcaggagaatggcgtgaacctgggaagcggaggttgcagtgagcctagatcgcaccactgcactccagcctgggccacaaagcaagtctcaaaaacaaaaacaaaaacaaaaaaatgattaacatttcaatcagtcaatgggtagactttgagtcacgctgattatccaccacaattgtgggcggagctcattcaataaactgaagacctttaagagaaaagactgaggtcccggccaggtgcggtggctcacgcctgtaatcccagcactttgggaggctgagccaggccaacatggtgaaacctcatctcggatacaaaaaattagccaggtgtggtggcgggcgcctgtgaccccagctacttgggaggctgaggcaggagaatcacttgaacctgggaggcggaggctgcagtgagcaaagatggcgccactgcactccagcctgggcaacaacagaaaaacaacaaaaatcatctcattttcatctgtgtcttccagtattaaagaggttgagtgtcatttctggcttactagccatttggatttcttctgatacacacttcatctcatttgcctaattttgtcgttgtcttcttattgctttctaagggctctctgtatactatggatattagtccttggttaatgacactgcaaatacttacaattttttttaatttttaattttcgtgggcacatagtttattgagaatttttttttttttgagatggcaggggtctcatatgttccccagactagagtgcagtggctattcacaggcgccgtctagcgcactacaaccttaaactcctgggctcaagcaattctcctgcctcagccttgggagtagctgggattacaagtgcccgccaccacgcctggtctgccaatactttctatcagtctgtcatgtttactgtcttttcctccatacagaagtttttccttctcagttgggtcaagtccattgacctttctgttacagcttgagttttgtgtcttacgtagaaaaggtgcccctgctctcactttctgcacagctatcaggtccagctcatagcagttcttctatttatccatccactgccccaggagctgcctgggcattcactgccccgcacccctctccagccccaaggtagagctcgggccctgggagtcccaggaccatcccggactggggagctgcttggtgtccagccccgggctcaagctcttctccagctctgcagctacctgaggggtagcagcccggatagcatcctggatgttggttaggtcccactgggtcctcaggagggcactgtctagcgtgaagaagccgtcgcgcgtgcgccgcacttgggtgcagacagcagtggtctttagttccaggccgatttcatgaaccaacttccgcagctctttctgcgtctcatgcatgcactgcacctctaagaggaattccggaggtgcaaagtagaggcatcggatgccagttatcagcatcggggacttgttcatgggccggatcaggcctctcacggccatctcataggcctcctgggtcttcaggtcgaggttggagtacatcaccagggccttctgatgggagccttggataacggccagaatgcggtccagcttctctctggtcacgtggtcataggttgtcttctctaccagcctcccgtcctcacggaagtcatctgtagctttgcccaggaggccacgcactgtgtaatccttggtaagatgagcattgtacatatcggtgaggagcctgcatccatgtcccacgccgagcaccatatgcactgaatctgactcatggttggagggggcctaggatccctgccaagctctccacaggattctgacaccaagtactccagaagcctgggcatccaaccgatgtcccacgccaaccttgagatgggcgaatgctggtccacataccagtggatggttgatgaaagagggtacgctggtggctgtgagggtcagctccttctcttcgctgccttccatggggcccagcaagaagcgaacacgctgtttaggagcgggaggcttcctggcattgagacccttcagaagttgtagctccactgtatcccgcaggtgcttccattttagccccgggggcttatagaccgcgaaaagcccatgcagccgcgacaagccagcagaccccatacttgaagatcacagcacccgctggacctggacggaagt

SEQ ID NO: 16147 - RNA, 1774 nt, Homo sapiens
  source 1..1774: mol_type = other RNA
gctgggattacaggcatgagccgccacacctggcccttattaaagttctgatcacacctggcccagtccctgacatccttcagcaatgttagttctgcttcctcctgcccctgcccagggcgagggccccccagctgcgtgatggactctggaagggcaagtgcaaattaaagatgagatgcttaattcttcccactgaaaataagggaagagaccttccccttcttccttttctacttcaaaaattttagctgtatgtaaatcacactccatcctccggtgttctggaagaaggtgggcctgactgcagctgtcctctgactccacaagcagaacctccctactgtaatgggttggatccactttgctatatgaaagagaggttttgttctgcctgctgtctctgtagtgagttgcccatcatgtgcatcatattctggtccaatgcttacttgataacacaattgttttccttcacttctactttcgtagggaagttttctgagagaagattttgtttttcattttaattccccagtagctcccataagacagggagagatgaactccactcccatctgtcttgtgtggaaatggtttcagacttctctgctggcttctttagttggagagtgggctgggcagcggggctgagagctgttaagggttgagggctgggggaaggcatgttttccagcactttccctctaacaaaccctgtaagatccagacaggacaaatctccagtccgagatgatgaacttctcccggatttggccagcgaatttcctgcctgacttggcacagtatatctctccttccacactccggatggaaatgttcttgaggtgactgtcagagatctggactttgtcacacatctcctggaagagcttcacacctccctggtccaggagcacacaaacgaacaccccacgcttgttggctgcctctagaatgtcacagaagatctccacatccgtgaacacatccatcaggatgaccaggacctggctagtccgggtgatgcagcggcggacgaggtctctgatgttgttgtgcttgacggtctggaagtacacagtggcgctggatttttccttcaggtagggcttctcagctgaggcccagctgtgcagtagggccggctcgctgccctctgaggccacagggaagtaggtgccggactgtagggagctggagtccagtcccttagggcctgcttccgcccctcccagggtgtctgggggacacgggggctccctggcctgggcctggatgtactgggcctccaccgaggacaagaagtccacctcgccttcctggctgagcacccgccagtaggcttcagaacccccatccaagagggcgtccgtggccagccgggcactctcgttgtcactaaagtcagccctggctggccggacccactggctcttgacatcttccagacgcttccggattttgcccaggtgccttgaccggctcatgcctcccgtccctgggtggtgctgggggaggctggcacgtcagctcctccagatgtgggaagcaaatggaacacaccacggaggagtggggctcccgcacccccgggaggccgcctgctcccaggaccggcgtgcagggcacctccaagaagtgatttaccgctgtcctgagcaatgcttctcagaactcctcatctgcagctgcgggattggcttatctctcagggccacctgccctgccctcgggccgggagggctggctcagacacctccttggcacagtc

SEQ ID NO: 16148 - RNA, 1039 nt, Homo sapiens
  source 1..1039: mol_type = other RNA
gctgggattacaggcatgagccgccacactcggcctaaacggttaatttttatagtctcttcctgagttgtataagggtaggtagaattttaatatccttatgtactaatgaaggaattgaggttaaacagtcagaaaacaaatgtcattgtgaactgcaagcaaaatgccactctccctgactaagaatttacattgccagagtaggctgttgcctagggaaccatgtcagaaaaaggtccagcatctcagaggactcacggtatgttgttctaggcttctgtcacgaatttttggtgtgtagaaccctacaaagcataatgtagaatcagtgagagccctgagcttgttttcctgcaactggatggtcccatctccatgggaaaagctttgaaattaaccgtgtgctcagaaccacgctggttttctcttccccagtgaaatctcacttcgtacagttcaaattcatgcccttgaggcaatggtcctcccgaaagaactgattttgacttcaggataacctgaatggtatgtccatcattggtgacttcacagtctcggcacaccacataatttggggagaggcggacatccaacagcgaggggtcatacctagcctctcttgagtttaggttaataggagactggtattccccattagcatcaggaaacaccagaccccactcaacaccttcctcgtagccccactccacaccctcctcttcttcctcctcatcctcttccttctcggggaaggcgacggtatcttcgatgaagctcaggtccgccatgggaaggccgcggggcccctcggcgctctcggcagcagtgcctgcgccttcgctgggcgcggggctggagccggagcggagcgcgcgtgggggagtgtgagcacgcgtgagcggcagtgtgagtgcgagagcgcctccgggtgtgaaccgcagtgtgagtgcaagcaggcgtgcgttcggaccgagtgttccagagacccgcgtgggaagcgcgtccggaggccccagcagagcgagggagcggctgt

SEQ ID NO: 16149 - RNA, 2099 nt, Homo sapiens
  source 1..2099: mol_type = other RNA
gctgggattacaggcatgagccgccacgcccagctgagattacattactttgagtgtttaatttcactatgacaggaagtagcctaatacatacttttttgtgttaattttctggattcatcctgatttttagtcttcgtacctgagtacaacaataaaggaaatcacttcttagatacattaaaattacttctaaacttgccccccacacatgaactgttttcagtttgctatttttaatggcccatgcttatttatatagacatagcataacactgctaacactttatggcctactgtcctctttcttagtattatattataaaatatttttctatatttccacatagttattgactcattttaatggctgcaaaatcaggtactcatttaagctcaaatggtttagtatcactcctcagaaatgtattcctccttctcttgattggtagtcataatcaaatgaagtgacattattctttgtagctggttacttacatttcaaatacactcatgagtggagccaaaactccattagttcattagtctggaagcactattaaatctccattaaaatgtcttcacttttcaattttgtgtgtgtgtgtgtgtgtgtggatggagtcttactctgttgcccaggctggagtgcagtggtgtgatctctgctcactgcaacttctgcctcctgggttcaagcgattctccatgcctcagcctcccaagtagctggaattacaggcatgtggcaccacacccagctaatttttgtatttgtagtagagacgaggtttcaccatgttggccaggctggtgtcgaacccctgacctcaggtgatccacccaccttggcctctcaaagtgctacgattacaggcatgagccactgcgcctggcccatttttcgatttttaacatgaggattaagtagactactacgcacatttgctaaaggcagccccttacatttctttttaagcagaaaatacttggtggttagagacagcagcgtcacagcataaccacctctaggctgtcagtgtgccctctaaaacaacagctgcacctcctctaatgtcaacccttccgtctggacgaagggaaattcccagctctcctcctcggtgggaacactgaaaagcatgcatttctttcttccccagatgctgggaccagtagctgctgagaacagcgtgtgcagaccctgtcactgggtcttcagccacaccaacccacggtgcaaaatatcttgagtaaaagtcaaatgcttgggtctgcccaccaggctctcctttaagggtaagaataagccctttcaccttccctgtgttttcaacttgcagcagattctccgtgttcactttcaggttctccagaaacgacctgttgtaaacgtcactgaggcggacgaggagcttttgggtatctggagaataacagatgtcctggaccagtgtgttgcctatggcagtctttatcaagtcctctacttcatggaagtcctgggggtgggctggataaagaggcaagtccaggacgatgccatcctctgctcgtctggcccttagttctccactcagagtgacaaacgtgagcgtgctattcatgttttttattttgtgaaacagcacagctgcagaagccagggtggcatggccacagagtgggacctcactcgctggtgtaaaccatctcagtccaaagcaggaactttgtgcaaagttgtctgtcgggtgcagttttcggataaaagcagtttcagagaggttcatctcccttgcaattttctgatgcatgtcttcatccaattcattttctaggaggcaaacagcagcaggattcccacgaaatgctcttgctgtgaatgcatctgctatgaaaataggaagcttcattttccttgcaagctgtttttgcaagttctcaaaattgctggtagcctgctttacgtcttctgggctgacgggactgcgagtgacttctgacgcagattcccaagatgagagaggctggagctgggggaggaaagccaatggcgacgaaggtgctcaactcccaaatccaggacaaaggaggcagacggcctcctttgtaattct

SEQ ID NO: 16150 - RNA, 2125 nt, Homo sapiens
  source 1..2125: mol_type = other RNA
gctgggattacaggcatgagccgccacgcccagctgagattacattactttgagtgtttaatttcactatgacaggaagtagcctaatacatacttttttgtgttaattttctggattcatcctgatttttagtcttcgtacctgagtacaacaataaaggaaatcacttcttagatacattaaaattacttctaaacttgccccccacacatgaactgttttcagtttgctatttttaatggcccatgcttatttatatagacatagcataacactgctaacactttatggcctactgtcctctttcttagtattatattataaaatatttttctatatttccacatagttattgactcattttaatggctgcaaaatcaggtactcatttaagctcaaatggtttagtatcactcctcagaaatgtattcctccttctcttgattggtagtcataatcaaatgaagtgacattattctttgtagctggttacttacatttcaaatacactcatgagtggagccaaaactccattagttcattagtctggaagcactattaaatctccattaaaatgtcttcacttttcaattttgtgtgtgtgtgtgtgtgtgtggatggagtcttactctgttgcccaggctggagtgcagtggtgtgatctctgctcactgcaacttctgcctcctgggttcaagcgattctccatgcctcagcctcccaagtagctggaattacaggcatgtggcaccacacccagctaatttttgtatttgtagtagagacgaggtttcaccatgttggccaggctggtgtcgaacccctgacctcaggtgatccacccaccttggcctctcaaagtgctacgattacaggcatgagccactgcgcctggcccatttttcgatttttaacatgaggattaagtagactactacgcacatttgctaaaggcagccccttacatttctttttaagcagaaaatacttggtggttagagacagcagcgtcacagcataaccacctctaggctgtcagtgtgccctctaaaacaacagctgcacctcctctaatgtcaacccttccgtctggacgaagggaaattcccagctctcctcctcggtgggaacactgaaaagcatgcatttctttcttccccagatgctgggaccagtagctgctgagaacagcgtgtgcagaccctgtcactgggtcttcagccacaccaacccacggtgcaaaatatcttgagtaaaagtcaaatgcttgggtctgcccaccaggctctcctttaagggtaagaataagccctttcaccttccctgtgttttcaacttgcagcagattctccgtgttcactttcaggttctccagaaacgacctgttgtaaacgtcactgaggcggacgaggagcttttgggtatctggagaataacagatgtcctggaccagtgtgttgcctatggcagtctttatcaagtcctctacttcatggaagtcctgggggtgggctggataaagaggcaagtccaggacgatgccatcctctgctcgtctggcccttagttctccactcagagtgacaaacgtgagcgtgctattcatgttttttattttgtgaaacagcacagctgcagaagccagggtggcatggccacagagtgggacctcactcgctggtgtaaaccatctcagtccaaagcaggaactttgtgcaaagttgtctgtcgggtgcagttttcggataaaagcagtttcagagaggttcatctcccttgcaattttctgatgcatgtcttcatccaattcattttctaggaggcaaacagcagcaggattcccacgaaatgctcttgctgtgaatgcatctgctatgaaaataggaagcttcattttccttgcaagctgtttttgcaagttctcaaaattgctggtagcctgctttacgtcttcttctgggctgacgggactgcgagtgacttctgacgcagattcccaagatgagagaggctggagctgggggaggaaagccaatggcgacgaaggtgctcaactcccaaatccaggacaaaggaggcagacggcctcctttgtaattctgccgcccggtggcgaagggtttt

SEQ ID NO: 16151 - RNA, 2066 nt, Homo sapiens
  source 1..2066: mol_type = other RNA
gctgggattacaggcatgagccgccacgcccagctgagattacattactttgagtgtttaatttcactatgacaggaagtagcctaatacatacttttttgtgttaattttctggattcatcctgatttttagtcttcgtacctgagtacaacaataaaggaaatcacttcttagatacattaaaattacttctaaacttgccccccacacatgaactgttttcagtttgctatttttaatggcccatgcttatttatatagacatagcataacactgctaacactttatggcctactgtcctctttcttagtattatattataaaatatttttctatatttccacatagttattgactcattttaatggctgcaaaatcaggtactcatttaagctcaaatggtttagtatcactcctcagaaatgtattcctccttctcttgattggtagtcataatcaaatgaagtgacattattctttgtagctggttacttacatttcaaatacactcatgagtggagccaaaactccattagttcattagtctggaagcactattaaatctccattaaaatgtcttcacttttcaattttgtgtgtgtgtgtgtgtgtgtggatggagtcttactctgttgcccaggctggagtgcagtggtgtgatctctgctcactgcaacttctgcctcctgggttcaagcgattctccatgcctcagcctcccaagtagctggaattacaggcatgtggcaccacacccagctaatttttgtatttgtagtagagacgaggtttcaccatgttggccaggctggtgtcgaacccctgacctcaggtgatccacccaccttggcctctcaaagtgctacgattacaggcatgagccactgcgcctggcccatttttcgatttttaacatgaggattaagtagactactacgcacatttgctaaaggcagccccttacatttctttttaagcagaaaatacttggtggttagagacagcagcgtcacagcataaccacctctaggctgtcagtgtgccctctaaaacaacagctgcacctcctctaatgtcaacccttccgtctggacgaagggaaattcccagctctcctcctcggtgggaacactgaaaagcatgcatttctttcttccccagatgctgggaccagtagctgtcactgggtcttcagccacaccaacccacggtgcaaaatatcttgagtaaaagtcaaatgcttgggtctgcccaccaggctctcctttaagggtaagaataagccctttcaccttccctgtgttttcaacttgcagcagattctccgtgttcactttcaggttctccagaaacgacctgttgtaaacgtcactgaggcggacgaggagcttttgggtatctggagaataacagatgtcctggaccagtgtgttgcctatggcagtctttatcaagtcctctacttcatggaagtcctgggggtgggctggataaagaggcaagtccaggacgatgccatcctctgctcgtctggcccttagttctccactcagagtgacaaacgtgagcgtgctattcatgttttttattttgtgaaacagcacagctgcagaagccagggtggcatggccacagagtgggacctcactcgctggtgtaaaccatctcagtccaaagcaggaactttgtgcaaagttgtctgtcgggtgcagttttcggataaaagcagtttcagagaggttcatctcccttgcaattttctgatgcatgtcttcatccaattcattttctaggaggcaaacagcagcaggattcccacgaaatgctcttgctgtgaatgcatctgctatgaaaataggaagcttcattttccttgcaagctgtttttgcaagttctcaaaattgctggtagcctgctttacgtcttctgggctgacgggactgcgagtgacttctgacgcagattcccaagatgagagaggctggagctgggggaggaaagccaatggcgacgaaggtgctcaactcccaaatccaggacaaaggaggcagacggcctccttt

SEQ ID NO: 16152 - RNA, 2100 nt, Homo sapiens
  source 1..2100: mol_type = other RNA
gctgggattacaggcatgagccgccacgcccagctgagattacattactttgagtgtttaatttcactatgacaggaagtagcctaatacatacttttttgtgttaattttctggattcatcctgatttttagtcttcgtacctgagtacaacaataaaggaaatcacttcttagatacattaaaattacttctaaacttgccccccacacatgaactgttttcagtttgctatttttaatggcccatgcttatttatatagacatagcataacactgctaacactttatggcctactgtcctctttcttagtattatattataaaatatttttctatatttccacatagttattgactcattttaatggctgcaaaatcaggtactcatttaagctcaaatggtttagtatcactcctcagaaatgtattcctccttctcttgattggtagtcataatcaaatgaagtgacattattctttgtagctggttacttacatttcaaatacactcatgagtggagccaaaactccattagttcattagtctggaagcactattaaatctccattaaaatgtcttcacttttcaattttgtgtgtgtgtgtgtgtgtgtggatggagtcttactctgttgcccaggctggagtgcagtggtgtgatctctgctcactgcaacttctgcctcctgggttcaagcgattctccatgcctcagcctcccaagtagctggaattacaggcatgtggcaccacacccagctaatttttgtatttgtagtagagacgaggtttcaccatgttggccaggctggtgtcgaacccctgacctcaggtgatccacccaccttggcctctcaaagtgctacgattacaggcatgagccactgcgcctggcccatttttcgatttttaacatgaggattaagtagactactacgcacatttgctaaaggcagccccttacatttctttttaagcagaaaatacttggtggttagagacagcagcgtcacagcataaccacctctaggctgtcagtgtgccctctaaaacaacagctgcacctcctctaatgtcaacccttccgtctggacgaagggaaattcccagctctcctcctcggtgggaacactgaaaagcatgcatttctttcttccccagatgctgggaccagtagctgtcactgggtcttcagccacaccaacccacggtgcaaaatatcttgagtaaaagtcaaatgcttgggtctgcccaccaggctctcctttaagggtaagaataagccctttcaccttccctgtgttttcaacttgcagcagattctccgtgttcactttcaggttctccagaaacgacctgttgtaaacgtcactgaggcggacgaggagcttttgggtatctggagaataacagatgtcctggaccagtgtgttgcctatggcagtctttatcaagtcctctacttcatggaagtcctgggggtgggctggataaagaggcaagtccaggacgatgccatcctctgctcgtctggcccttagttctccactcagagtgacaaacgtgagcgtgctattcatgttttttattttgtgaaacagcacagctgcagaagccagggtggcatggccacagagtgggacctcactcgctggtgtaaaccatctcagtccaaagcaggaactttgtgcaaagttgtctgtcgggtgcagttttcggataaaagcagtttcagagaggttcatctcccttgcaattttctgatgcatgtcttcatccaattcattttctaggaggcaaacagcagcaggattcccacgaaatgctcttgctgtgaatgcatctgctatgaaaataggaagcttcattttccttgcaagctgtttttgcaagttctcaaaattgctggtagcctgctttacgtcttcttctgggctgacgggactgcgagtgacttctgacgcagattcccaagatgagagaggctggagctgggggaggaaagccaatggcgacgaaggtgctcaactcccaaatccaggacaaaggaggcagacggcctcctttgtaattctgccgcccggtggcgaagggtttt

SEQ ID NO: 16153 - RNA, 5007 nt, Homo sapiens
  source 1..5007: mol_type = other RNA
gctgggattacaggcatgagccgccatatctggcctatttattttttaatttttcaaatgagaaggttgggttaggtaatttttaaaaatcgcttcaagtttcttaactccacaattattttcctgagactcttgcaagcaactgatctttataggtcatgcctcaaattcccaattgatgtcatctgggcaaatcagtccaatgacagccacaagtggtcagaaagctttcttagcagccctcttggtcactaggcacactacctaggagtcaagctgtgacaagaggctgcttcttaaacttacaaaagataggatcttccaggatgtgctgctctgatgtttttgaagggcatagagaaacacacgggcaatgtttgcagaggcaacagactaaagaaagcacatctatagttgtattggctttgtgtgggttgtatggtaaacaggtagtcaccctgcttaatgtgggtatcccattttccataaatgtctatttcaccaccccaaaaagccctcttatcatgaaattaatcatctgatgcacttcaagtaccagtcacaaaaatgatgaactcaggcagaattccactgctagacaagcccagacaaaaactgttactgttagccaaggaaatttgcacacaattttgataagtggcactaaagccacataagacaggaaatgggttagaggacatcaatgtattgagacagaaagtgaaagggtgggcaggatttgcgaggttaccagtttgaatatggccattcctgcttttactaaaggtcaatttagaatacaaatgttacagaattcatttagagccaaaaagtaattctgacaaagactgtcttaaaatgcaagatttttaggtccaaaatttcttacgtaacctaaaaaatggaaatcttcacaatgtaatgagattgggtcatttaaatagtgttatatctaaccagtccagacagaccagctaaacaatcctattattaaaagcctctagagagtgttcaacaaactccttagataatgaagcttggggcagcaacacatccctcattatagtcagaaagttctcttaacatgtgagccaggttattgcgtgcatttatgttttcccacatgctgctctttcctcaaggaatgcgattctcctccccgactccctgcctggttcgctcattcttcaagatcaaacacaaaagtcactgtgtgtgtgatgcttctccaattccactcatcctggctgccattcatgcactagtgcatgtatgcatttttacattttttaaattacaaaaatcaacctattataactgcttagatatatatgaagtaaaaatgaaagttctccctttacatgacccatcccccatcatttccctctttatcttatactgtcagcattcccagcttgtagcacagtgtctggcaatagtaaatcctcaaaaaatgatcaatgaataatttaataatgattaataaataaattaatgatgatggtgaagataaatttttagcatttattgaacgctaactacaaaccagggagtgtgttaaatattttataaaaatcaatgaatgagctaaaatgccattctgttatttttttgtataggttttaatattttactcataaatatgcttaaagaatattataattatatgacttagattgtaaaacaatatgtacagcagtgtcctattttttagaataaaattataaatatgtgctcacatatgtgtttgtgcatgcatagaaaacagattagaaaggaatatattctaacaccattatctctagctggtagaattatggaaaatttttatttccttctttttgcttctaaattttatataatgagcatatttggctttgtataatcatttttaaaaagttgttttagaagaatagtactgatatatcattcccttttagcagttttctctaggataaaaaataagaggaagtctgagcttaactaattaaaaaaacagatttctttaaaaaatattagcaaatcattagtgttcttactggagaaagggcagtgttcaaagaagaattaaacaaatcattccagttgcaggaaaaattcaatttactgcatgcagactgtttcttgactgaaaagttaattcctttcattcagaatcagtatgcatattcactggctatatttcatctcacatctgcaaacttaatttttcctttcttggtcatcagaagattaggaaataaattttagtccaggcaatagatcctacttggcaagctcaaaataactcaattattaaaaagcagcacacaaagaccagtagtgacttccaaaggattgttaacaatacttaaaaaaaaaaaaaaaaaaagaaaaagaaaaaagggtccaactgtctaaaagaagactagagatacatgaataagaaaatacgatgttttggaattatgtgcaaaatagtaatgctgcatattacccatcctttaagttttagcaataattagaaaaaatagtttcccaacaataaaagttataaaataatgtcatcatatcacctagaagagattatagatttttataaacaaaatatgtgttattatgaatatttgtatgtactctccaagaactaaaagatgaagttcccctttcaggatcccctgtgcctgagaaggaaactttccagtgaaagcctactagctagttaaaaatttcttaaaaaagaaaatcttcttagttgtatacttgggagcatcctttctcttgggcggatccctgttagacatatacaacttttaatgtttgcacctttaagtgtagggatggtctctgagtatgcccacattcgtatctaagatattcaatgcctgtccttcagacacttaacaaggactctgagttccaaatctcccttgagtgctgcagtgcatgctgacgctctttaaaagccatagcactcccttactgtgaaataaaactgctctgtctcttgctggttggctctcctcttagcaatgctgggcttgctcatgaaggtttcagagaccgtggacttgacggactccatggagttgctgtactggaagcagtcagacacatcaaagtcctcgacagtcacaatgtcctggatggtttgcagggtggcctccattgtcttctttacctcttcgttttcaatctttagagtggataagcgagactgcagttgttggcatctctgtaccagctcactctggacaggctgctgggcacagagctgggaagccatatcccccatgtggggctgaaactcaaacttcataggggggcagaagacgttgttgtacatctccatgaggcgctgcttgtcactggtggcatccaggttttctactgcattctcgatggcatccagaccctcatgcttcgactgttccaggtttaactcagcagagaggaaggtgcgtagagcccggttcagacttgcatggtagcctaagtcacaacaatcaataaggtcagataggtcatggatgtagtacttgaagacagatgcattggttgcctccaaagccagcaagtactcattctgggctttgatggccttcagcttattctccgtgtacttggcttggtgcttctccttcatcttctcaatcttcttcactgagctcctccggacatgtttctcctcaatgcgaacgttggccgtggagtcaggggagcatggggtctgccggtcctcctgctttaccgatttaccaatttgcttctcctcctgcttctccgcctcctttagtttgctctgagcactgatgctgtcggcattgtacatgtgatatgtcttcatgaccgagtagagctcgttcaggaccttcatcaaatcatcttggagctgctggccgacttctttactctttttaaagagtcttcctgagtcctcgctgacttgtacaaatcgaggaatgatattattcaggtagatgtcactcagggtggtatggtccctgctttcccacttcacctggtttaagaggagattccagcagttgactggagagagaacattctgatccttcttgaattgctggtccttggtgctgcgtgtcttggccaggaagtgttctgccagcttctccaggttgcgggagtagtccatctcaatctctgccttctttcggaagaagtcctggaggtcctgcaacagttgcacccgaagctcacactgctggtccaggcatttcatctgctctgtgagctgagcacggatctctttgacctgagtatcgtactctgctatgatctccttatcctttttgaatttggctggagacgtcatgttttccttctttcttccaaattcgaattgtgaattgatagatccacggaaaaaatccaaccacctaaatcaatacctccaagaccgcttctctcgagggcagaaggggccccccacggtggtctccagcgctccgtggagcgcgggctgcgggctgggcagacggctacggcgggcacatgcagacggtgggcgctgaggccgggtgcggcggcggctggtgcctgtgctagagccggagccgcagcctcagcattagccgggagaactgcagcgcccggaggctggcctggggtctgacatcaacgacacaggcggggagtggaagtccttccgcacaacatggtgtggggctgcgggggtgtggacgcgcccagctgtgtccccgggagggagtgggtgcttttcggggtgccgggggagggctgggcgtgcttcgcggttttttgtcgtagaggctcaaagatgctgcaaatcaaatcccaaacgggagccgcaacagcgcagactggatcggaagtcgtttgctccggttcacttgcctggctctgacgcgacgggtcccaggcccccggttccgcttcccactcagagctctcctcccctctcttccccgccacccgtttctacgcagatcggtgccccagtccctggaggagcctccgccgcctccgccaactccgcaggacccc

SEQ ID NO: 16154 - RNA, 5010 nt, Homo sapiens
  source 1..5010: mol_type = other RNA
gctgggattacaggcatgagccgccatatctggcctatttattttttaatttttcaaatgagaaggttgggttaggtaatttttaaaaatcgcttcaagtttcttaactccacaattattttcctgagactcttgcaagcaactgatctttataggtcatgcctcaaattcccaattgatgtcatctgggcaaatcagtccaatgacagccacaagtggtcagaaagctttcttagcagccctcttggtcactaggcacactacctaggagtcaagctgtgacaagaggctgcttcttaaacttacaaaagataggatcttccaggatgtgctgctctgatgtttttgaagggcatagagaaacacacgggcaatgtttgcagaggcaacagactaaagaaagcacatctatagttgtattggctttgtgtgggttgtatggtaaacaggtagtcaccctgcttaatgtgggtatcccattttccataaatgtctatttcaccaccccaaaaagccctcttatcatgaaattaatcatctgatgcacttcaagtaccagtcacaaaaatgatgaactcaggcagaattccactgctagacaagcccagacaaaaactgttactgttagccaaggaaatttgcacacaattttgataagtggcactaaagccacataagacaggaaatgggttagaggacatcaatgtattgagacagaaagtgaaagggtgggcaggatttgcgaggttaccagtttgaatatggccattcctgcttttactaaaggtcaatttagaatacaaatgttacagaattcatttagagccaaaaagtaattctgacaaagactgtcttaaaatgcaagatttttaggtccaaaatttcttacgtaacctaaaaaatggaaatcttcacaatgtaatgagattgggtcatttaaatagtgttatatctaaccagtccagacagaccagctaaacaatcctattattaaaagcctctagagagtgttcaacaaactccttagataatgaagcttggggcagcaacacatccctcattatagtcagaaagttctcttaacatgtgagccaggttattgcgtgcatttatgttttcccacatgctgctctttcctcaaggaatgcgattctcctccccgactccctgcctggttcgctcattcttcaagatcaaacacaaaagtcactgtgtgtgtgatgcttctccaattccactcatcctggctgccattcatgcactagtgcatgtatgcatttttacattttttaaattacaaaaatcaacctattataactgcttagatatatatgaagtaaaaatgaaagttctccctttacatgacccatcccccatcatttccctctttatcttatactgtcagcattcccagcttgtagcacagtgtctggcaatagtaaatcctcaaaaaatgatcaatgaataatttaataatgattaataaataaattaatgatgatggtgaagataaatttttagcatttattgaacgctaactacaaaccagggagtgtgttaaatattttataaaaatcaatgaatgagctaaaatgccattctgttatttttttgtataggttttaatattttactcataaatatgcttaaagaatattataattatatgacttagattgtaaaacaatatgtacagcagtgtcctattttttagaataaaattataaatatgtgctcacatatgtgtttgtgcatgcatagaaaacagattagaaaggaatatattctaacaccattatctctagctggtagaattatggaaaatttttatttccttctttttgcttctaaattttatataatgagcatatttggctttgtataatcatttttaaaaagttgttttagaagaatagtactgatatatcattcccttttagcagttttctctaggataaaaaataagaggaagtctgagcttaactaattaaaaaaacagatttctttaaaaaatattagcaaatcattagtgttcttactggagaaagggcagtgttcaaagaagaattaaacaaatcattccagttgcaggaaaaattcaatttactgcatgcagactgtttcttgactgaaaagttaattcctttcattcagaatcagtatgcatattcactggctatatttcatctcacatctgcaaacttaatttttcctttcttggtcatcagaagattaggaaataaattttagtccaggcaatagatcctacttggcaagctcaaaataactcaattattaaaaagcagcacacaaagaccagtagtgacttccaaaggattgttaacaatacttaaaaaaaaaaaaaaaaaaagaaaaagaaaaaagggtccaactgtctaaaagaagactagagatacatgaataagaaaatacgatgttttggaattatgtgcaaaatagtaatgctgcatattacccatcctttaagttttagcaataattagaaaaaatagtttcccaacaataaaagttataaaataatgtcatcatatcacctagaagagattatagatttttataaacaaaatatgtgttattatgaatatttgtatgtactctccaagaactaaaagatgaagttcccctttcaggatcccctgtgcctgagaaggaaactttccagtgaaagcctactagctagttaaaaatttcttaaaaaagaaaatcttcttagttgtatacttgggagcatcctttctcttgggcggatccctgttagacatatacaacttttaatgtttgcacctttaagtgtagggatggtctctgagtatgcccacattcgtatctaagatattcaatgcctgtccttcagacacttaacaaggactctgagttccaaatctcccttgagtgctgcagtgcatgctgacgctctttaaaagccatagcactcccttactgtgaaataaaactgctctgtctcttgctggttggctctcctcttagcaatgctgggcttgctcatgaaggtttcagagaccgtggacttgacggactccatggagttgctgtactggaagcagtcagacacatcaaagtcctcgacagtcacaatgtcctggatggtttgcagggtggcctccattgtcttctttacctcttcgttttcaatctttagagtggataagcgagactgcagttgttggcatctctgtaccagctcactctggacaggctgctgggcacagagctgggaagccatatcccccatgtggggctgaaactcaaacttcataggggggcagaagacgttgttgtacatctccatgaggcgctgcttgtcactggtggcatccaggttttctactgcattctcgatggcatccagaccctcatgcttcgactgttccaggtttaactcagcagagaggaaggtgcgtagagcccggttcagacttgcatggtagcctaagtcacaacactgatcaataaggtcagataggtcatggatgtagtacttgaagacagatgcattggttgcctccaaagccagcaagtactcattctgggctttgatggccttcagcttattctccgtgtacttggcttggtgcttctccttcatcttctcaatcttcttcactgagctcctccggacatgtttctcctcaatgcgaacgttggccgtggagtcaggggagcatggggtctgccggtcctcctgctttaccgatttaccaatttgcttctcctcctgcttctccgcctcctttagtttgctctgagcactgatgctgtcggcattgtacatgtgatatgtcttcatgaccgagtagagctcgttcaggaccttcatcaaatcatcttggagctgctggccgacttctttactctttttaaagagtcttcctgagtcctcgctgacttgtacaaatcgaggaatgatattattcaggtagatgtcactcagggtggtatggtccctgctttcccacttcacctggtttaagaggagattccagcagttgactggagagagaacattctgatccttcttgaattgctggtccttggtgctgcgtgtcttggccaggaagtgttctgccagcttctccaggttgcgggagtagtccatctcaatctctgccttctttcggaagaagtcctggaggtcctgcaacagttgcacccgaagctcacactgctggtccaggcatttcatctgctctgtgagctgagcacggatctctttgacctgagtatcgtactctgctatgatctccttatcctttttgaatttggctggagacgtcatgttttccttctttcttccaaattcgaattgtgaattgatagatccacggaaaaaatccaaccacctaaatcaatacctccaagaccgcttctctcgagggcagaaggggccccccacggtggtctccagcgctccgtggagcgcgggctgcgggctgggcagacggctacggcgggcacatgcagacggtgggcgctgaggccgggtgcggcggcggctggtgcctgtgctagagccggagccgcagcctcagcattagccgggagaactgcagcgcccggaggctggcctggggtctgacatcaacgacacaggcggggagtggaagtccttccgcacaacatggtgtggggctgcgggggtgtggacgcgcccagctgtgtccccgggagggagtgggtgcttttcggggtgccgggggagggctgggcgtgcttcgcggttttttgtcgtagaggctcaaagatgctgcaaatcaaatcccaaacgggagccgcaacagcgcagactggatcggaagtcgtttgctccggttcacttgcctggctctgacgcgacgggtcccaggcccccggttccgcttcccactcagagctctcctcccctctcttccccgccacccgtttctacgcagatcggtgccccagtccctggaggagcctccgccgcctccgccaactccgcaggacccc

SEQ ID NO: 16155 - RNA, 1235 nt, Homo sapiens
  source 1..1235: mol_type = other RNA
gctgggattacaggcatgagccgccgcgccctgcctgattcttaacaattctgagtatactctcagaagctgggttagagtcccaggcttcttttgaaaagtacctcctaggctggaagttcttgctggctccttgttctgattagaattcattccctgacccctggaaaattttgtttcctggctcctcacgacatctttctattctctctatttgagcctgtttctctcacaggaacttctcagtcaaccgaaacccctgttcctccaatcctgcgtcaccacgatggtcccaatactggccgggttctttctccgcggcagaagtttactgaagatcttgaattacaatggccctctggggctcctcggatatccccaaattaatccacctttttccaagtggccaggcagcaccgcttcaagaagtctctccgtgcttgaagtctgcaggcaccagtaccctcagacgccctccctcctgccaagatgccctagagcaagttccccgcagctgaaggggcagcgaaggaagagccgaagtgaagactggtgaggttatcagctaaaaccgccccttatttcttttgctctctgtcagagctaccggctaccaccaggagcttgtcaggtgaacatcaaaagacagagggggaaaaatggtagttgcctgtaatcccagctattcgagaggctgaggcaggagaatcgcttgaacctgggaggcagaggtttcagtgagccgagatcgcgccactgcactccagcctggatacttattgagattatagcagaaccctccatttgagctacatctgtccacttctgctctgattcatccatgcctgtgcacatctggaaggccttggagcagttcccgccagaaatctgtttgcatgagtcaatgaagagcctcctgagagaaaattgatcaagactgcaggtttactacaagggccagaactcaggaagagccggatggaagcgatgcacgggacaaggtctgtgggaaggggcgcggagcttccatgccctctgggcgcgccaccatttccaggacctccgtgtgttcaccagaccggaagctctggtttttacggaggctcattacttagtcatgattgattaaaccactggccattggaaattaatgcaatctccagcccccagtcctcccctggaggtggaagttggaagctgggaagcgggctgtggacacgatttgtaatgaatgc

SEQ ID NO: 16156 - RNA, 2629 nt, Homo sapiens
  source 1..2629: mol_type = other RNA
gctgggattacaggcatgagccgccgcgcctggccccaagtgttttacttctgtggcctcaattgcttagtaaaagtcgtcagcactgtgctcagcactgtgaaaagtttaagcttctccagaaaggatacaactttgttcttagtttcttcagaactgagacactgtggaactatctcttcatgatttgttccctcagcgaactgagtaaacgcctccaaggtatgttgttctagcagccaactcctgtcagctagcagtaaggcaaacatacaggacaggttgggcagaattctgtcctggatagcttcaggtataaaaagttttcctaaagaagatacaaaatccaacattgccaaacgaacatagtcaggaagctctaatttaagtagcgaggtctgcaaagttactgcctgaagtatcagtttaggatctagagtttgaatgaaaaatcccaacagtggaagtaaaaggctgaatgtctgttgaacataaggttgatctgctacctgtttaatgtttaaaaaagcccaaagctgactcacaacttcgataattgcagtttgttttcctgtatccaaagcttcaccagcagaattacatactgcaagcaaagcagacagtactgtgttcagagattctagttctcccaaagtacgactcctgctcagccatttcctgcattctgcagtgcctactgtggtgacctcatggacagtttgttccctaagctcaggaggtaacgcctggaaggaaatatgttgccacagaggcagattttctgcttcttttggggaaaatttctggataaactccagctgatggggtggtgccatgaagaaaaagagacgcttcaacagtattgataggttgatgagttgataacattctccagggcatgactttatcagatgagccactatggtgacatggtgtgcacacagttcagcagtcccatatcgagcaaggaagcaccatgcatccatagctaacaaagaggtgatcatattagcactaagtacagcattcagcagagcagcatccagttcagcaaacagtgagggatgaaaggaagtaataaatgtacacagatgaacacaaacatgctgatacaaggtgacagccacctcagctttccccttactctttaatccctgtaaatgaacaggtagagagagttcaccagaacactgctcaaaactgtagaaaacggctttgagtagagatatcctggttgtcgtttctgagacctggctgtctgtgcaccacagggtttgcacttccttaggctgagatggcagcttatccatgacaacaaccagaagaagacattgtggaaactgcagttcacatggcaggtctaatttactgtccaaaaccacctgcatgaaaggctgaaatgtgagcagctgactgataagtggatccagtgtcactaggaaagcacctgctatttcctcttggtgtgctttagaaatcctggtagcataaaggcttggaggaaacttgctgtgtatctgaagatacagttggtgcaaagtacagcaagaatcagagaggaaaggaagaaattccttagcgtagtgcaaaagggagttggcaaaaaaacgacacaatttgagtgttttctgaaataatctgtagtcagcattatcctgtgcatctgactgtgtcatctgctcagctaactgtaaacaagaatggaaggagaaaagaatgtcttcacacaagctagtaattatatctttgtgtttcaactggctttttattatggactggtgcttaaggctctgcttaattataaacttccaagtattggcatgaaatgcatggtccatactggaaataacagagcagatatccaataaagaatgaataactattaccatattcaaaatatcatcattgtcatctactaaagggtccatgcaaaccatgtccagcagttccattaactgcttttgaagagaataggcctccttgaaaagagcctggagaaggtctgaaactaggtgtaaacacccagaatacacagattcactattcttacaatgcacaaatgtgcttttaattatatgaaggactgaggaggggagactctgaatattttccaaaatgatggattcctgtgtggcacagatatgctgaacacatcctgtgagagctcctaagagctgcaccattgtttgtaaaatattccttagagtggtctggatttccaaattttggcttgacagtcctctggcttgactggttaattcatacatcatgtcatcgaataatttcacagtctttggtaacacttgtgaaaagaaagtctgttccaatgtcaggtggttcatatgaggtaaaaacatttctacaataattttcaaaatttgaatatgctcaatccaactgtcagaatgttgagacaatgagaggagtcggggcaggacggacggcagttcccggcggcatagctcctctggccagctacttaattcttccaggggaaccgcgctagctgggaccgcaccttcctgagacatactttcgtcaaacaggagagcttcaaaccagacccgccaaagcccagaccggaaactcgcagtcccgccaacccttgcgcgctctccgccggctccaa

SEQ ID NO: 16157 - RNA, 3912 nt, Homo sapiens
  source 1..3912: mol_type = other RNA
gctgggattacaggcatgagccgccgcggccggcaatttttgtattttaagtggagatgaggtttcaccatgttagccaggctggtcttcagctcctgacctcaggtgatccatccgccttggtctcccaaaatgctgggattacaggcatgagccactgtgctcggcctgcaggttttaacaagaggagcatgaactatcattttgacacaaagacagcttaaaaaaaataataaagctggctggacgcggtggctcacacctgtaatcccagcactttgggaggctgaggtgggtggatcacaaggtcaggagatcaagaccatcctggacaacatggtgaaaccccgtctccactaaaaacacaaaattagccaggcatggtggcaggcgcctgtaatcccagctactcaggagggtgagccaggagaatcacttgaactcgggaggcagagcttgtagtgagcagagatcgcaccactgcactccagcctgggcaacagagtgagactccatctcaaaaaaaaaaaaaaaaaaaaaaaaaaaaagactatttgttgaatgttgaaaggaggagctaaaatcagttgaaattcggagtagaaggaaaactggagtgtctcattcacttcactctgatttgaatttttttttttttttgagacaagagtattgctctgtcacacaggctggagtacaatggtgcgatatcagctcactgcaatcttcgcctcctgggttcaagtgattctcctgcctcagcctcctgagtagctaggattacaggcatgcgccaccacacccagctaattcttgtattttttagtagaaatggggttttaccatgttggccaggctggtctcgaactcctgacctcaggtgatctgcccacctcgacctcccaaagtgctgggattacaggcgtgagccaccatgcccggcctgattttttttttttttttttttttgaggcagggtcttgctctgtcccccaggctggagtgcagtggcatactcatggctcactgcagcctccaattcctaaactccaatgatcttctcacctcagcctgccaagtagctaggattacagatgtgtgccgccatgctaatttttaaaaattttttgtatagatgggttctcactatgagcccaggctcatcttgaagttctgggctcaagcaatcctcttaccttggctttccaaagtactgggattacaggcgggagccaccatgccagccgtcactctcatttttgagcacaggaattgtgcccaaaggctaggataaggaattaaagatgcatgccaagaaatacccacaaacattaattataaaagggagactatactaatgtttgtgaaaagcttatactaacatagagcaatatttaagttataaagttaaatgaaaaagggtataaaactgtatgaacagtacaatctcaactatgtaaaaaccaaccaaaatctgccctaaaaaggctggaaggaaatagctcaaaatgttaatgtgattgtatttaagaagtgtatctaatagggatcttttttcttcctttttagttttctgtcttttccaaatgtttctctactggggagatttttttaaaaagctattagggaaggagtagaacaaaagtggaaaaaaaaatctattagttacaaaaaactgagtctgatagaagcattgaatttgagttaatgaatctaagtctagcctataagaatttgtacatttagaaaactatgaaacagtccaggctactccatgaatccattggtaggaccagaggctggaggtggaagtgccacctggtcctgcctgataaaaaatgctgaatcagccaggcacggtggcccacacacctgtaatcccaccattttgggaggctgaggtgggcggatcacctgaggtcaggagtttgaaaccagcctggccaacatgacgaaacactgtctctactaaaagtacaaaaattggccagcgtggtggcaggcgcctgtaatcccagctactcaggaggattacgtgaacccaggaggcagaggttgcagtgagccgagatggcgccactgcactccagcctgggtgacaagagtgagactccatctcaaaaaaacaaaacaaaacaaaacaacaacaacaaaaaaacccaaatcaatcaggaatgtcacatatttacaaaaaggaacagaaatactcacatttagcaaaaacttatttgtccattaatactataatcaaacatgcagattttctcgtattttctgtgcggatggcaagttacaaaaatgctattatcacaactgtagaatgtcaatcctagtttagaaacagtaataaaacagcacttcaacaagagtggaccgagaaagtgcacgacttagaaaattataaaaaatgcttcctacaaaaatgattccctttaagacatttgttcactgtacacattttaaggtcccctctcccaccccccaacaaaaatagaggcagaacctctaagcactttctaacaaagtgtcccctggtttgttcctctgacaaaccctgactgaaggctcatgatgtgcaggcactggggtctcaaagaggagaaagacttgtccctgcctcacggatgcctcagtcttcccaaagcaggaggcagacaagtcaccaaccgctacggatgtagaatggatgtattatacatccattaaaagcagatgccaatgccttcttaaaattaaacgatatgctgcaattcccactgaattacttatacaaacctccttacatacaagctgtcctgacttactaggaagcaaaaatgccaccaccttctcctgataaatacttctctaatgggcaggcattaaattacattttgtgatgtttgcccctaaacatcacaatgcctagtgaagtcagttaactttcttttaagcaatggtgcctattttactctgagaatgagacactttgaaactaaggaaggaaccagtcctgtatctagatcaagactcatcagtaccatcaaaagctgagatgaaacagtgtaagtttcaacagaaatcttcaatctcccatccgttgatgtgcaatgcgctcctgtgtcagccgctccaggtctttctgcacatttgggtggtcttccagatcttcgtagagcgacctgacgatgtccagtctcctgtaattctcaggcttgactaggctccggacaacctggaggcatcgctctttcagagtatacactagggttggctagttcctactccatcctgctctcttccttctccgggaagtgctccttaactgaaaccacacaaccgcaacccctccatctcccagcaggcaggtaagtcaatttcccacgccacacacggtcggctcttccggcgccaacatgaccctggcttgttcctgtctttgcatctgtcagtctccccaggaggaatgtgttctccacgagggcagggactacgcagaactggcccactggagtcatgaggactcggtagctgtggatgcggcggcccgtgccaggcggcagcgttgggtagggctgcggctcgccgtcgaagttgagccatacgggcagcacgacgcgcggactgcgattgcagaagatgacctgggagggctcgcgcgagttcaccgagcgcagcacgggccgcggccgcccggcctccatctcctcctcggcgcccagttcctccgggccggactcttccgggccggactcctcggcgcccgactcctccccgccgtcttcttcagggccgtactcttcgacgcctgcctcctccgcgcctacctcggcctcgtcccagttctccgccctccggggcattccctccgcgatccagaccacccgggccggacgccgcgggatccgcgggtcggacgcggggcggagctgc

SEQ ID NO: 16158 - RNA, 3653 nt, Homo sapiens
  source 1..3653: mol_type = other RNA
gctgggattacaggcatgagccgccgcggccggcaatttttgtattttaagtggagatgaggtttcaccatgttagccaggctggtcttcagctcctgacctcaggtgatccatccgccttggtctcccaaaatgctgggattacaggcatgagccactgtgctcggcctgcaggttttaacaagaggagcatgaactatcattttgacacaaagacagcttaaaaaaaataataaagctggctggacgcggtggctcacacctgtaatcccagcactttgggaggctgaggtgggtggatcacaaggtcaggagatcaagaccatcctggacaacatggtgaaaccccgtctccactaaaaacacaaaattagccaggcatggtggcaggcgcctgtaatcccagctactcaggagggtgagccaggagaatcacttgaactcgggaggcagagcttgtagtgagcagagatcgcaccactgcactccagcctgggcaacagagtgagactccatctcaaaaaaaaaaaaaaaaaaaaaaaaaaaaagactatttgttgaatgttgaaaggaggagctaaaatcagttgaaattcggagtagaaggaaaactggagtgtctcattcacttcactctgatttgaatttttttttttttttgagacaagagtattgctctgtcacacaggctggagtacaatggtgcgatatcagctcactgcaatcttcgcctcctgggttcaagtgattctcctgcctcagcctcctgagtagctaggattacaggcatgcgccaccacacccagctaattcttgtattttttagtagaaatggggttttaccatgttggccaggctggtctcgaactcctgacctcaggtgatctgcccacctcgacctcccaaagtgctgggattacaggcgtgagccaccatgcccggcctgattttttttttttttttttttttgaggcagggtcttgctctgtcccccaggctggagtgcagtggcatactcatggctcactgcagcctccaattcctaaactccaatgatcttctcacctcagcctgccaagtagctaggattacagatgtgtgccgccatgctaatttttaaaaattttttgtatagatgggttctcactatgagcccaggctcatcttgaagttctgggctcaagcaatcctcttaccttggctttccaaagtactgggattacaggcgggagccaccatgccagccgtcactctcatttttgagcacaggaattgtgcccaaaggctaggataaggaattaaagatgcatgccaagaaatacccacaaacattaattataaaagggagactatactaatgtttgtgaaaagcttatactaacatagagcaatatttaagttataaagttaaatgaaaaagggtataaaactgtatgaacagtacaatctcaactatgtaaaaaccaaccaaaatctgccctaaaaaggctggaaggaaatagctcaaaatgttaatgtgattgtatttaagaagtgtatctaatagggatcttttttcttcctttttagttttctgtcttttccaaatgtttctctactggggagatttttttaaaaagctattagggaaggagtagaacaaaagtggaaaaaaaaatctattagttacaaaaaactgagtctgatagaagcattgaatttgagttaatgaatctaagtctagcctataagaatttgtacatttagaaaactatgaaacagtccaggctactccatgaatccattggtaggaccagaggctggaggtggaagtgccacctggtcctgcctgataaaaaatgctgaatcagccaggcacggtggcccacacacctgtaatcccaccattttgggaggctgaggtgggcggatcacctgaggtcaggagtttgaaaccagcctggccaacatgacgaaacactgtctctactaaaagtacaaaaattggccagcgtggtggcaggcgcctgtaatcccagctactcaggaggattacgtgaacccaggaggcagaggttgcagtgagccgagatggcgccactgcactccagcctgggtgacaagagtgagactccatctcaaaaaaacaaaacaaaacaaaacaacaacaacaaaaaaacccaaatcaatcaggaatgtcacatatttacaaaaaggaacagaaatactcacatttagcaaaaacttatttgtccattaatactataatcaaacatgcagattttctcgtattttctgtgcggatggcaagttacaaaaatgctattatcacaactgtagaatgtcaatcctagtttagaaacagtaataaaacagcacttcaacaagagtggaccgagaaagtgcacgacttagaaaattataaaaaatgcttcctacaaaaatgattccctttaagacatttgttcactgtacacattttaaggtcccctctcccaccccccaacaaaaatagaggcagaacctctaagcactttctaacaaagtgtcccctggtttgttcctctgacaaaccctgactgaaggctcatgatgtgcaggcactggggtctcaaagaggagaaagacttgtccctgcctcacggatgcctcagtcttcccaaagcaggaggcagacaagtcaccaaccgctacggatgtagaatggatgtattatacatccattaaaagcagatgccaatgccttcttaaaattaaacgatatgctgcaattcccactgaattacttatacaaacctccttacatacaagctgtcctgacttactaggaagcaaaaatgccaccaccttctcctgataaatacttctctaatgggcaggcattaaattacattttgtgatgtttgcccctaaacatcacaatgcctagtgaagtcagttaactttcttttaagcaatggtgcctattttactctgagaatgagacactttgaaactaaggaaggaaccagtcctgtatctagatcaagactcatcagtaccatcaaaagctgagatgaaacagtgtaagtttcaacagaaatcttcaatctcccatccgttgatgtgcaatgcgctcctgtgtcagccgctccaggtctttctgcacatttgggtggtcttccagatcttcgtagagcgacctgacgatgtccagtctcctgtaattctcaggcttgactaggctccggacaacctggaggcatcgctctttcagagtatacactcggtagctgtggatgcggcggcccgtgccaggcggcagcgttgggtagggctgcggctcgccgtcgaagttgagccatacgggcagcacgacgcgcggactgcgattgcagaagatgacctgggagggctcgcgcgagttcaccgagcgcagcacgggccgcggccgcccggcctccatctcctcctcggcgcccagttcctccgggccggactcttccgggccggactcctcggcgcccgactcctccccgccgtcttcttcagggccgtactcttcgacgcctgcctcctccgcgcctacctcggcctcgtcccagttctccgccctccggggcattccctccgcgatccagaccacccgggccggacgccgcgggatccgcgggtcggacgcggggcggagctgc

SEQ ID NO: 16159 - RNA, 3776 nt, Homo sapiens
  source 1..3776: mol_type = other RNA
gctgggattacaggcatgagccgccgcggccggcaatttttgtattttaagtggagatgaggtttcaccatgttagccaggctggtcttcagctcctgacctcaggtgatccatccgccttggtctcccaaaatgctgggattacaggcatgagccactgtgctcggcctgcaggttttaacaagaggagcatgaactatcattttgacacaaagacagcttaaaaaaaataataaagctggctggacgcggtggctcacacctgtaatcccagcactttgggaggctgaggtgggtggatcacaaggtcaggagatcaagaccatcctggacaacatggtgaaaccccgtctccactaaaaacacaaaattagccaggcatggtggcaggcgcctgtaatcccagctactcaggagggtgagccaggagaatcacttgaactcgggaggcagagcttgtagtgagcagagatcgcaccactgcactccagcctgggcaacagagtgagactccatctcaaaaaaaaaaaaaaaaaaaaaaaaaaaaagactatttgttgaatgttgaaaggaggagctaaaatcagttgaaattcggagtagaaggaaaactggagtgtctcattcacttcactctgatttgaatttttttttttttttgagacaagagtattgctctgtcacacaggctggagtacaatggtgcgatatcagctcactgcaatcttcgcctcctgggttcaagtgattctcctgcctcagcctcctgagtagctaggattacaggcatgcgccaccacacccagctaattcttgtattttttagtagaaatggggttttaccatgttggccaggctggtctcgaactcctgacctcaggtgatctgcccacctcgacctcccaaagtgctgggattacaggcgtgagccaccatgcccggcctgattttttttttttttttttttttgaggcagggtcttgctctgtcccccaggctggagtgcagtggcatactcatggctcactgcagcctccaattcctaaactccaatgatcttctcacctcagcctgccaagtagctaggattacagatgtgtgccgccatgctaatttttaaaaattttttgtatagatgggttctcactatgagcccaggctcatcttgaagttctgggctcaagcaatcctcttaccttggctttccaaagtactgggattacaggcgggagccaccatgccagccgtcactctcatttttgagcacaggaattgtgcccaaaggctaggataaggaattaaagatgcatgccaagaaatacccacaaacattaattataaaagggagactatactaatgtttgtgaaaagcttatactaacatagagcaatatttaagttataaagttaaatgaaaaagggtataaaactgtatgaacagtacaatctcaactatgtaaaaaccaaccaaaatctgccctaaaaaggctggaaggaaatagctcaaaatgttaatgtgattgtatttaagaagtgtatctaatagggatcttttttcttcctttttagttttctgtcttttccaaatgtttctctactggggagatttttttaaaaagctattagggaaggagtagaacaaaagtggaaaaaaaaatctattagttacaaaaaactgagtctgatagaagcattgaatttgagttaatgaatctaagtctagcctataagaatttgtacatttagaaaactatgaaacagtccaggctactccatgaatccattggtaggaccagaggctggaggtggaagtgccacctggtcctgcctgataaaaaatgctgaatcagccaggcacggtggcccacacacctgtaatcccaccattttgggaggctgaggtgggcggatcacctgaggtcaggagtttgaaaccagcctggccaacatgacgaaacactgtctctactaaaagtacaaaaattggccagcgtggtggcaggcgcctgtaatcccagctactcaggaggattacgtgaacccaggaggcagaggttgcagtgagccgagatggcgccactgcactccagcctgggtgacaagagtgagactccatctcaaaaaaacaaaacaaaacaaaacaacaacaacaaaaaaacccaaatcaatcaggaatgtcacatatttacaaaaaggaacagaaatactcacatttagcaaaaacttatttgtccattaatactataatcaaacatgcagattttctcgtattttctgtgcggatggcaagttacaaaaatgctattatcacaactgtagaatgtcaatcctagtttagaaacagtaataaaacagcacttcaacaagagtggaccgagaaagtgcacgacttagaaaattataaaaaatgcttcctacaaaaatgattccctttaagacatttgttcactgtacacattttaaggtcccctctcccaccccccaacaaaaatagaggcagaacctctaagcactttctaacaaagtgtcccctggtttgttcctctgacaaaccctgactgaaggctcatgatgtgcaggcactggggtctcaaagaggagaaagacttgtccctgcctcacggatgcctcagtcttcccaaagcaggaggcagacaagtcaccaaccgctacggatgtagaatggatgtattatacatccattaaaagcagatgccaatgccttcttaaaattaaacgatatgctgcaattcccactgaattacttatacaaacctccttacatacaagctgtcctgacttactaggaagcaaaaatgccaccaccttctcctgataaatacttctctaatgggcaggcattaaattacattttgtgatgtttgcccctaaacatcacaatgcctagtgaagtcagttaactttcttttaagcaatggtgcctattttactctgagaatgagacactttgaaactaaggaaggaaccagtcctgtatctagatcaagactcatcagtaccatcaaaagctgagatgaaacagtgtaagtttcaacagaaatcttcaatctcccatccgttgatgtgcaatgcgctcctgtgtcagccgctccaggtctttctgcacatttgggtggtcttccagatcttcgtagagcgacctgacgatgtccagtctcctgtaattctcaggcttgactaggctccggacaacctggaggcatcgctctttcagagtatacactggcagtgtgatattggcaaaaataggctgtccgtcaacattgagagatggcacaaataattcagtttggttaaccagaagcccatcgtgtgtccctgcatctctgaagagccaaaggtgacctcggtagctgtggatgcggcggcccgtgccaggcggcagcgttgggtagggctgcggctcgccgtcgaagttgagccatacgggcagcacgacgcgcggactgcgattgcagaagatgacctgggagggctcgcgcgagttcaccgagcgcagcacgggccgcggccgcccggcctccatctcctcctcggcgcccagttcctccgggccggactcttccgggccggactcctcggcgcccgactcctccccgccgtcttcttcagggccgtactcttcgacgcctgcctcctccgcgcctacctcggcctcgtcccagttctccgccctccggggcattccctccgcgatccagaccacccgggccggacgccgcgggatccgcgggtcggacgcggggcggagctgc

SEQ ID NO: 16160 - RNA, 2220 nt, Homo sapiens
  source 1..2220: mol_type = other RNA
gctgggattacaggcatgagccgccgctcctggccagtaacttcttactttacaaacaacacaatacattttaacttgacatttgctttatcctatataatacaaacataacaaaatacatttaaaatgttgttgaaatatacaaaaatttaatgtaatttttgcgtctgagatgtttaaataagaaacttctttaatcaggtatccctttggactgcaagagcagtttatatcatagctttgcagcataatctttttactctcaggctcttcaagcatttttatcttctttgaaacttctatctaaacaaaaatagtattaaaaaagataacagaaggggttagattctgccaatgaactgtggacatcagtatctcattcttctatttgcctccttattctagtttgaaaaagctttggaacacattattacctatcattattacatatttcttgtagctttagtgttactcccccgactggaaatagaagttgctctttaataaggcccagggtgcttagggagcaatgcgagatttttcttacatctcttgggccaaccctatacaactaattctgggaaagggattgttataatacactgtccttgaaaagtttctttcagtccatttggagaaatgttggataaagataacttagtgcttacaagtgctctattattagtagtataataacaataattattattaaactaaaagttatctattactttatcaccctttctcaatttatgttttctcactctttaaaacatttaccccaacagggtgaaaataatggtttaaaaattgtaccttcatttacctttattatactacctaattgcccataggacatctagctctcacagttttgtcattagaagcaaaggacctgccaaatttctgaaccttttaaaaagagaaaataaatgccacaagcattttctattttagttttggaaatgttcttttttttttgtataaagggggaaaaattaaaaaaaaaaacctctcccctgaaaatatttgatgttttctatctgaatataaatcctgcagaagtcatctaagcctccaagtatctgtttccttcttggttaatagcacaacctggatgtcagacaggctgaccatgactcacagtgggactctaggcaactagtgtcaataggcttggggaccacaatgagtgaaaacaaaaacccttcctcttccattgtgtgttctaagagtgagcagacctaagagtggtggtttaagcactttctatcagaatggtgattgcttcagtgttctcaaggagatggcaacatcatggaagggcagcaacgtgagtcagcaacgtggtatatgggtcccaatcagcatctgcttctgatttgtttttgaaagaaaatccttagtcggttttcatttgaagcctgctgcagatcacagcgtcagggaaacattccaccttgctcctgggccagagcattccttggcaagaaagatctatttaaagatgaacgaccgagatcggatcgtgccttccccttggttgagctgttttcttatttgtgacaatttccagcgtaatatcttgatccactcatcagcttctactccggtctttgcacagagataaaatgtcctgaatggaaataccaaacaaaaacagtttaccctttcttgtgaataatcgaattgtacagctgaacattctgttaggtctaggatccgaattggttctggtgacatctggtctttgaagtatttcagttcattcctgtgcagagtaaaccatcttgttttccaggtcttgaccaggcctccctgtttggtgaggtaaccttctttggtgcccagagaaggtgctgtgggcacaaggtcatcttctgttcttcctgtctgcattgctgtgtgaacccggacagattcataaatggagggttcttccacttttcttgggtagggatgttttagaaccatcagagtgccctctagaccctgcagggtgaggctgggcctgggtggggtctggctgagagcagtggcctgaaatatccaattctagtccttgtcattctggtaatctgaagttgagagccctgggaggggcttgtccattgtgtggacaaatgcttttcctggtgatgttaatcaaacataagctataagaaatatctgtacttctggcgtgaacccgggaggcggagcttgcagtgggccgagatc

SEQ ID NO: 16161 - RNA, 2427 nt, Homo sapiens
  source 1..2427: mol_type = other RNA
gctgggattacaggcatgagccgccgctcctggccagtaacttcttactttacaaacaacacaatacattttaacttgacatttgctttatcctatataatacaaacataacaaaatacatttaaaatgttgttgaaatatacaaaaatttaatgtaatttttgcgtctgagatgtttaaataagaaacttctttaatcaggtatccctttggactgcaagagcagtttatatcatagctttgcagcataatctttttactctcaggctcttcaagcatttttatcttctttgaaacttctatctaaacaaaaatagtattaaaaaagataacagaaggggttagattctgccaatgaactgtggacatcagtatctcattcttctatttgcctccttattctagtttgaaaaagctttggaacacattattacctatcattattacatatttcttgtagctttagtgttactcccccgactggaaatagaagttgctctttaataaggcccagggtgcttagggagcaatgcgagatttttcttacatctcttgggccaaccctatacaactaattctgggaaagggattgttataatacactgtccttgaaaagtttctttcagtccatttggagaaatgttggataaagataacttagtgcttacaagtgctctattattagtagtataataacaataattattattaaactaaaagttatctattactttatcaccctttctcaatttatgttttctcactctttaaaacatttaccccaacagggtgaaaataatggtttaaaaattgtaccttcatttacctttattatactacctaattgcccataggacatctagctctcacagttttgtcattagaagcaaaggacctgccaaatttctgaaccttttaaaaagagaaaataaatgccacaagcattttctattttagttttggaaatgttcttttttttttgtataaagggggaaaaattaaaaaaaaaaacctctcccctgaaaatatttgatgttttctatctgaatataaatcctgcagaagtcatctaagcctccaagtatctgtttccttcttggttaatagcacaacctggatgtcagacaggctgaccatgactcacagtgggactctaggcaactagtgtcaataggcttggggaccacaatgagtgaaaacaaaaacccttcctcttccattgtgtgttctaagagtgagcagacctaagagtggtggtttaagcactttctatcagaatggtgattgcttcagtgttctcaaggagatggcaacatcatggaagggcagcaacgtgagtcagcaacgtggtatatgggtcccaatcagcatctgcttctgatttgtttttgaaagaaaatccttagtcggttttcatttgaagcctgctgcagatcacagcgtcagggaaacattccaccttgctcctgggccagagcattccttggcaagaaagatctatttaaagatgaacgaccgagatcggatcgtgccttccccttggttgagctgttttcttatttgtgacaatttccagcgtaatatcttgatccactcatcagcttctactccggtctttgcacagagataaaatgtcctgaatggaaataccaaacaaaaacagtttaccctttcttgtgaataatcgaattgtacagctgaacattctgttaggtctaggatccgaattggttctggtgacatctggtctttgaagtatttcagttcattcctgtgcagagtaaaccatcttgttttccaggtcttgaccaggcctccctgtttggtgaggtaaccttctttggtgcccagagaaggtgctgtgggcacaaggtcatcttctgttcttcctgtctgcattgctgtgtgaacccggacagattcataaatggagggttcttccacttttcttgggtagggatgttttagaaccatcagagtgcctgtctcgcttccaatcaaaggctgatttgcaaaatgcttgacaaaatccttcaaagatgagaattcattaaagccaaatttaaatgaatatccagtatattcaacatgaaagtgtttaacagaatctttggccctcacagagagagagtacagcccggtggtctcattgctgtccctcagaaggtagctgccgtcacatccatttgagaggagaagagcttcagcagcatggcgtgtgaggttgccgtgataccaccccaagtcctggagcagctcagcctctccatcggatctgctccacagatctgagggatcctgggtgctcatcttcccttctagaagttctgctctgcccattcgcgcccttcacagaggtagagagagagacacaactgggctgctcctgacaccttctcgctctgtgagacagcagcctgctatggc

SEQ ID NO: 16162 - RNA, 2465 nt, Homo sapiens
  source 1..2465: mol_type = other RNA
gctgggattacaggcatgagccgccgctcctggccagtaacttcttactttacaaacaacacaatacattttaacttgacatttgctttatcctatataatacaaacataacaaaatacatttaaaatgttgttgaaatatacaaaaatttaatgtaatttttgcgtctgagatgtttaaataagaaacttctttaatcaggtatccctttggactgcaagagcagtttatatcatagctttgcagcataatctttttactctcaggctcttcaagcatttttatcttctttgaaacttctatctaaacaaaaatagtattaaaaaagataacagaaggggttagattctgccaatgaactgtggacatcagtatctcattcttctatttgcctccttattctagtttgaaaaagctttggaacacattattacctatcattattacatatttcttgtagctttagtgttactcccccgactggaaatagaagttgctctttaataaggcccagggtgcttagggagcaatgcgagatttttcttacatctcttgggccaaccctatacaactaattctgggaaagggattgttataatacactgtccttgaaaagtttctttcagtccatttggagaaatgttggataaagataacttagtgcttacaagtgctctattattagtagtataataacaataattattattaaactaaaagttatctattactttatcaccctttctcaatttatgttttctcactctttaaaacatttaccccaacagggtgaaaataatggtttaaaaattgtaccttcatttacctttattatactacctaattgcccataggacatctagctctcacagttttgtcattagaagcaaaggacctgccaaatttctgaaccttttaaaaagagaaaataaatgccacaagcattttctattttagttttggaaatgttcttttttttttgtataaagggggaaaaattaaaaaaaaaaacctctcccctgaaaatatttgatgttttctatctgaatataaatcctgcagaagtcatctaagcctccaagtatctgtttccttcttggttaatagcacaacctggatgtcagacaggctgaccatgactcacagtgggactctaggcaactagtgtcaataggcttggggaccacaatgagtgaaaacaaaaacccttcctcttccattgtgtgttctaagagtgagcagacctaagagtggtggtttaagcactttctatcagaatggtgattgcttcagtgttctcaaggagatggcaacatcatggaagggcagcaacgtgagtcagcaacgtggtatatgggtcccaatcagcatctgcttctgatttgtttttgaaagaaaatccttagtcggttttcatttgaagcctgctgcagatcacagcgtcagggaaacattccaccttgctcctgggccagagcattccttggcaagaaagatctatttaaagatgaacgaccgagatcggatcgtgccttccccttggttgagctgttttcttatttgtgacaatttccagcgtaatatcttgatccactcatcagcttctactccggtctttgcacagagataaaatgtcctgaatggaaataccaaacttgaagtgctggtatatatgcacctactcctgccagcaaacaaaaacagtttaccctttcttgtgaataatcgaattgtacagctgaacattctgttaggtctaggatccgaattggttctggtgacatctggtctttgaagtatttcagttcattcctgtgcagagtaaaccatcttgttttccaggtcttgaccaggcctccctgtttggtgaggtaaccttctttggtgcccagagaaggtgctgtgggcacaaggtcatcttctgttcttcctgtctgcattgctgtgtgaacccggacagattcataaatggagggttcttccacttttcttgggtagggatgttttagaaccatcagagtgcctgtctcgcttccaatcaaaggctgatttgcaaaatgcttgacaaaatccttcaaagatgagaattcattaaagccaaatttaaatgaatatccagtatattcaacatgaaagtgtttaacagaatctttggccctcacagagagagagtacagcccggtggtctcattgctgtccctcagaaggtagctgccgtcacatccatttgagaggagaagagcttcagcagcatggcgtgtgaggttgccgtgataccaccccaagtcctggagcagctcagcctctccatcggatctgctccacagatctgagggatcctgggtgctcatcttcccttctagaagttctgctctgcccattcgcgcccttcacagaggtagagagagagacacaactgggctgctcctgacaccttctcgctctgtgagacagcagcctgctat

SEQ ID NO: 16163 - RNA, 2489 nt, Homo sapiens
  source 1..2489: mol_type = other RNA
gctgggattacaggcatgagccgccgctcctggccagtaacttcttactttacaaacaacacaatacattttaacttgacatttgctttatcctatataatacaaacataacaaaatacatttaaaatgttgttgaaatatacaaaaatttaatgtaatttttgcgtctgagatgtttaaataagaaacttctttaatcaggtatccctttggactgcaagagcagtttatatcatagctttgcagcataatctttttactctcaggctcttcaagcatttttatcttctttgaaacttctatctaaacaaaaatagtattaaaaaagataacagaaggggttagattctgccaatgaactgtggacatcagtatctcattcttctatttgcctccttattctagtttgaaaaagctttggaacacattattacctatcattattacatatttcttgtagctttagtgttactcccccgactggaaatagaagttgctctttaataaggcccagggtgcttagggagcaatgcgagatttttcttacatctcttgggccaaccctatacaactaattctgggaaagggattgttataatacactgtccttgaaaagtttctttcagtccatttggagaaatgttggataaagataacttagtgcttacaagtgctctattattagtagtataataacaataattattattaaactaaaagttatctattactttatcaccctttctcaatttatgttttctcactctttaaaacatttaccccaacagggtgaaaataatggtttaaaaattgtaccttcatttacctttattatactacctaattgcccataggacatctagctctcacagttttgtcattagaagcaaaggacctgccaaatttctgaaccttttaaaaagagaaaataaatgccacaagcattttctattttagttttggaaatgttcttttttttttgtataaagggggaaaaattaaaaaaaaaaacctctcccctgaaaatatttgatgttttctatctgaatataaatcctgcagaagtcatctaagcctccaagtatctgtttccttcttggttaatagcacaacctggatgtcagacaggctgaccatgactcacagtgggactctaggcaactagtgtcaataggcttggggaccacaatgagtgaaaacaaaaacccttcctcttccattgtgtgttctaagagtgagcagacctaagagtggtggtttaagcactttctatcagaatggtgattgcttcagtgttctcaaggagatggcaacatcatggaagggcagcaacgtgagtcagcaacgtggtatatgggtcccaatcagcatctgcttctgatttgtttttgaaagaaaatccttagtcggttttcatttgaagcctgctgcagatcacagcgtcagggaaacattccaccttgctcctgggccagagcattccttggcaagaaagatctatttaaagatgaacgaccgagatcggatcgtgccttccccttggttgagctgttttcttatttgtgatcagtcttctcctcgggagatatacagagagcagacaaaataaatcagcttttgtccttgaccaatttccagcgtaatatcttgatccactcatcagcttctactccggtctttgcacagagataaaatgtcctgaatggaaataccaaacaaaaacagtttaccctttcttgtgaataatcgaattgtacagctgaacattctgttaggtctaggatccgaattggttctggtgacatctggtctttgaagtatttcagttcattcctgtgcagagtaaaccatcttgttttccaggtcttgaccaggcctccctgtttggtgaggtaaccttctttggtgcccagagaaggtgctgtgggcacaaggtcatcttctgttcttcctgtctgcattgctgtgtgaacccggacagattcataaatggagggttcttccacttttcttgggtagggatgttttagaaccatcagagtgcctgtctcgcttccaatcaaaggctgatttgcaaaatgcttgacaaaatccttcaaagatgagaattcattaaagccaaatttaaatgaatatccagtatattcaacatgaaagtgtttaacagaatctttggccctcacagagagagagtacagcccggtggtctcattgctgtccctcagaaggtagctgccgtcacatccatttgagaggagaagagcttcagcagcatggcgtgtgaggttgccgtgataccaccccaagtcctggagcagctcagcctctccatcggatctgctccacagatctgagggatcctgggtgctcatcttcccttctagaagttctgctctgcccattcgcgcccttcacagaggtagagagagagacacaactgggctgctcctgacaccttctcgctctgtgagacagcagcctgctatggc

SEQ ID NO: 16164 - RNA, 2597 nt, Homo sapiens
  source 1..2597: mol_type = other RNA
gctgggattacaggcatgagccgccgctcctggccagtaacttcttactttacaaacaacacaatacattttaacttgacatttgctttatcctatataatacaaacataacaaaatacatttaaaatgttgttgaaatatacaaaaatttaatgtaatttttgcgtctgagatgtttaaataagaaacttctttaatcaggtatccctttggactgcaagagcagtttatatcatagctttgcagcataatctttttactctcaggctcttcaagcatttttatcttctttgaaacttctatctaaacaaaaatagtattaaaaaagataacagaaggggttagattctgccaatgaactgtggacatcagtatctcattcttctatttgcctccttattctagtttgaaaaagctttggaacacattattacctatcattattacatatttcttgtagctttagtgttactcccccgactggaaatagaagttgctctttaataaggcccagggtgcttagggagcaatgcgagatttttcttacatctcttgggccaaccctatacaactaattctgggaaagggattgttataatacactgtccttgaaaagtttctttcagtccatttggagaaatgttggataaagataacttagtgcttacaagtgctctattattagtagtataataacaataattattattaaactaaaagttatctattactttatcaccctttctcaatttatgttttctcactctttaaaacatttaccccaacagggtgaaaataatggtttaaaaattgtaccttcatttacctttattatactacctaattgcccataggacatctagctctcacagttttgtcattagaagcaaaggacctgccaaatttctgaaccttttaaaaagagaaaataaatgccacaagcattttctattttagttttggaaatgttcttttttttttgtataaagggggaaaaattaaaaaaaaaaacctctcccctgaaaatatttgatgttttctatctgaatataaatcctgcagaagtcatctaagcctccaagtatctgtttccttcttggttaatagcacaacctggatgtcagacaggctgaccatgactcacagtgggactctaggcaactagtgtcaataggcttggggaccacaatgagtgaaaacaaaaacccttcctcttccattgtgtgttctaagagtgagcagacctaagagtggtggtttaagcactttctatcagaatggtgattgcttcagtgttctcaaggagatggcaacatcatggaagggcagcaacgtgagtcagcaacgtggtatatgggtcccaatcagcatctgcttctgatttgtttttgaaagaaaatccttagtcggttttcatttgaagcctgctgcagatcacagcgtcagggaaacattccaccttgctcctgggccagagcattccttggcaagaaagatctatttaaagatgaacgaccgagatcggatcgtgccttccccttggttgagctgttttcttatttgtgatcagtcttctcctcgggagatatacagagagcagacaaaataaatcagcttttgtccttgaccaatttccagcgtaatatcttgatccactcatcagcttctactccggtctttgcacagagataaaatgtcctgaatggaaataccaaacttgaagtgctggtatatatgcacctactcctgccagcaaactgcagaaatgttaaggaagttgtagattcatattattattccaagtcagatgtatatactcgaataagacaaaaacagtttaccctttcttgtgaataatcgaattgtacagctgaacattctgttaggtctaggatccgaattggttctggtgacatctggtctttgaagtatttcagttcattcctgtgcagagtaaaccatcttgttttccaggtcttgaccaggcctccctgtttggtgaggtaaccttctttggtgcccagagaaggtgctgtgggcacaaggtcatcttctgttcttcctgtctgcattgctgtgtgaacccggacagattcataaatggagggttcttccacttttcttgggtagggatgttttagaaccatcagagtgcctgtctcgcttccaatcaaaggctgatttgcaaaatgcttgacaaaatccttcaaagatgagaattcattaaagccaaatttaaatgaatatccagtatattcaacatgaaagtgtttaacagaatctttggccctcacagagagagagtacagcccggtggtctcattgctgtccctcagaaggtagctgccgtcacatccatttgagaggagaagagcttcagcagcatggcgtgtgaggttgccgtgataccaccccaagtcctggagcagctcagcctctccatcggatctgctccacagatctgagggatcctgggtgctcatcttcccttctagaagttctgctctgcccattcgcgcccttcacagaggtagagagagagacacaactgggctgctcctgacaccttctcgctctgtgagacagcagcctgctat

SEQ ID NO: 16165 - RNA, 4724 nt, Homo sapiens
  source 1..4724: mol_type = other RNA
gctgggattacaggcatgagccgctgagcctggcttttttaatgtcttggaccaaaaaggacttgcttttcttcctggaggtatttggaaggagaaacagtgagaaatgaacgccagctcacataggcacctagctgccccgagatgactttagctcaaagtcagctgtgacataggtaaggaaccgagaaggttgggaggctgagaaagggctagacaacagatatttctgagctcccataggaaaagatgcccaaccaaaaccttgttcaaatcccagtgttccactttctgtgtgaccttgggcaagtatttaacatctctggacctccttcccccatctgtaaaatgtagagaatgtatcaggggcttggaatcgtgcctggcacatagtatatccaatatacatattttctttttctttttctttttcttttctttttttttttttgagacagggtcttgctctgtcacccaagctggagtacagtgatgcaatcacagctcactgcagccttgacctcccaggctcaagtgatcctcccacttcagcctcctgagtagctgggaccacaggtgcacaccaccaaacccagctaatttttgtattttttgtattttatgttgctgaggctggtcttgaacccctgggctcaggcaatcctcctgcctcggcctcccaaagtactacgatttgctaggattataggtgagagccactatgcccagcccctatgactttttttttttttttgagacagagtctctgtttcgcccaggctggagtacagtggtgtgatctcggcccactgcagccgccacctcccaggttcaagcaattctgtctcagcctcccaagtagctgggactacaggcatgtgccaccacacccagctaatttttgtatttttagtagagacggggtttcaccatgttggccaggctggtcttgaactcctgacctcaggtgatccacctgcctcggcctcacaaagtgctgggattacaggcgtgagccacctggcctgccccctatgacctcttgatacacccctgggtgtcccttttgccccacacacccaccatattctaaagcagcctcagcgtctccgctaaaacctgctctttctctcagggataactggccactctgtgggacattccctagccgcgtccctccagtctgtgggggctatggcctgtccacttggctcctgagtgtgcccgcactcacccctcctcccttccatggctcagcccaggcccatcgtctccctcttcattcctgcctcagcctcccacaggcacccagcctcagtacccgctctgctccacctctccagagcaactagggggatcatcctaaaacccaaacctaaccatgacccactcctactctaaacccttccatggctctctagggccctcaggaaagagaccaggttcccatgctggtcatttaaggacactaacgggtgctcgtgcgcacccctctgccctccttccctctttccctgcataccgttcatactaaactgcttgtcagaagctggtggccagcatgcttttccatctccaggcctttgcacacagctcctcccacctggtatgccctctccatgccttttctacttgtctactgttgggacccagctcaaatgccccagccctttttaaaatttttatttttgtagagatggggtcttgctatgttggccaggcttgtctcaaactcctagcctcaagtgatcttcccaccttggccttcccaaggtgctgggattacaggactgagccactgtgccccgcttctttccttcttttcttttctttctttcttttttttttttgagacggagtcttgctgtcacccaggttggatgcagtggcgcgatctcggctcattgcaggctccgcccccaccggggttcacgccattctcctgcctcagcctcccgagtagctgggactacaggcgcctgccacctcgcctggctaattttttgtatttttagtagagacagggtttcaccgtgttagccaggacttactttctttctttttctttttttctttcttacttttctttctttttcttttttctttcttacttttctttctttttctttctctctctctctctttctctttctttttccttccttccttccatctttccctttctttctttctttctttctctctctttctttctttctttctctctttctttcagacagggtctcactctgtcccgcaggctggagtgcagcagtgccatcataactcactgcagcctcaaactcctggcctcaagtgatccttccacctcagcctctgaagtagccaggatcacaggcatgcaccaccacacccagctaatttttagattttgtggttgttgttgagataaggcctcactgtgttgcctaggctagtctcaaactcctggcctcaagcgatcctccttcctcagccttccaaagtgctgggtgtataggcgtgagccaccacactcagcctgaaatccttttgaagttgtattatgatgatcaccattttacagataaggaaacaaaatcagagaggtagtgtgactgcccaaggacacaggccagacgtggctaagttgggatttgagctcaaccaggctgattccagggcacaacatacaaatgtggacagctcttacaatggtgtcatggttaagggcagcacctcccatgccattcagatctgggctggggtcctatgtctgtttcctgcctgccaggctgctgaggaagagtctatcgcccaggcctacaccaggggtccctccatgggtcctgctccctggagacacctgagaaaaatgagtcaggtacaacttcttcctgcctatttctcatagttcaggtcttagttcgatgtcccttcctctaggaagtcctccctgactttccaggctggattgggcctagtccctatgcttctccgacttcagccctgaccactctgcctgtgctttcaacacctcacctcctccattaaagtcctgaccattttgggccatcactgtctggggacaggtctgtccacctcactggactgcaagctccataagggcagttctccacccccaactatgtctccagcactgtctagcacagggccagcacacaggaggggtttaggggcaaattcttctattcttcccatttggcagctgaggaaatcaaggctcagagacgggcagtcacttgtccagggtgtagcgaccaatctggtgcctgaaatgaggtctgagcccacagcccagtagaatcagcagttgacgagtggttaattgagagacacagacggaacatgaaagagaatgagaaacagagacagcaagagggaaagacagaggcagcgagaatgccagagagccagagagacacagtgtaaagaggatgagagaaaggacagagaacaaggttatgttggtgcccagtggagcccgggacatggggacagggagtgctgcccttcacatcccagccagatgctgggaaacaaaggagagacggtggacggcaaggcctcaagatcacctgctgtgctcgtggacattcctgtacagccagctctggtcgcctggacccctcagtcccaggccaggcacacccaagcctggcagaggctgccccagctacctggggatggaagcgtagtcggtgtgggagctggcagagagttgctggtgcgactccggctgggggcccaggatgtccacccgatcgtcctcatccgcattgaaactggcagggcacggagggggcagcaggatgagctccgtgaggccgtggaggtcggacacgtggcggaaggtctgcagcaccagcaccatggccaccaggcccaggaagaggtagactgtgaccagcaccttgtagagggcccggtagggctggccaggggcctccccgggcacgtagtcgcccaggccgatggtggacagagagataaagcagaagtagaaggcatccaagaagctccaggcctcctcgaggtgggcaaagatcacagccggcaccagaaagcagacggtcactacgacccccaacagggccaccaagtgccagcaggccgcccgccgggggtcccagccccaacgcatgctcagccaagacaggggcacgtgagtcagcagcagtgacaggcgctgggctgaggcggtcagcagcagcatggtggtcggcacgcccaggagcgcaaaggcgatggagaaggccttgcccgcatcagtcagtggcgttgtgtacccatagcccacggtggtgatcagcgtgctggcgaagaagagagcagaggcgaagtcccaggcggggtccgaggcgttggcggaccccgaagcgttagcaagcacgacccgccccagccgtccggccgccagcactcgctccacgaaggcgtccagggcgggggcagccacacacgggctgcgctgaagcagctgcgcccgcagcgtctccagctcggctcggagcctggcttcgtgcggcccctccagccgcgccaccaacagcgcgcccagcaccaggtacgcggcgtacgcggccaaggcgcccgccagaagcgcgcccctccgcatggcacccaccgggaccccgcgagccctgggtggccccgctgacgtggcccccgcctccggaccgtctggcacctagttccagttccgggagtgctacaggcgcggc

SEQ ID NO: 16166 - RNA, 790 nt, Homo sapiens
  source 1..790: mol_type = other RNA
gctgggattacaggcatgagccgctgcacctggccataacatatttcttgtattccatatcccatacaattcacgcattgaaagtgtaatgcccagcggcttttagcgcattcacagagttgtgcgacgatgaccacaatcagttttagaacatttttcacctgctattttgatattcagattggcatccagaagtaaattttcagcttttaaatcacgatgaacaatgttccgacagtgacaaaaatagacagctgtgacgatctgtttgaacttccgacgtgcctccttttctgccattctaccatgggccaccaggtggtcaaatatttcccctccactagcatattctgtcaccagataaatcatccgttctgtctccataacctggtagagcctgatgatatgggggtggcaaagcatcttcataatttgaacttcccggaaaatcttcttcaagttttcttcatccagctgggtcttatctatgatcttgatagcaaccttggccttggtgacgaggtgcgtggcccgcttgaccaccgcgaagttgcccttgccgatggtgcggtcgatctcgtagtagccgatacgggcgggcatgggtccgcgggaggccggggctgggggacgcggctggccggccgcaggggacacggcagcgggggcggctggggaccccggcgcgggcggaggcagcaggcggcccgcgggcccggctcccccagtcccggccccggcagccccgccagctccgctcgccgccgccgccgccatcttgttgtgcagt

SEQ ID NO: 16167 - RNA, 679 nt, Homo sapiens
  source 1..679: mol_type = other RNA
gctgggattacaggcatgagccgctgtgcccagctcccatttgcatgttcttttccatattcctgattattaaatgtgtctgttcttaggatttcatttgaaccagttgtaacatctgcctggtttccttaaattggtttaggagtagaataaaatatttgacacatattctttttttaatatatgtatggaaggcatgattttgcctctttttgaagtgtcttttagaaggacgatagtgagaggctcaccgggcagaaggcacgcgtgcagaggcctggaggcttgctcttctcggctgctgagtagccagtagcctgacgcaaatccttatcagagcagaccacattttccagcccccgttcatgaagggtggagggagctgttgggaccggttctgagctcccatcagatcctctggagaactcctaggaatgcaggaggtggagctgaggggcagaggccagagctggactcctttccctgcactggatggtcagcgggccctttcctgaacgccaggcctcttgcagggcctacgtaggggctcctactgcggcttcttccctggcagagcccagcaggagctcctcggctcccctagctctgcttcctcttttgatttgcataacaatctgcccagacgagctttgtacctctgcatcagggctggagccca

SEQ ID NO: 16168 - RNA, 1161 nt, Homo sapiens
  source 1..1161: mol_type = other RNA
gctgggattacaggcatgagccgctgtgcccagtctccttcctgaagctttgaatttatgttactagcaaaccaaacaatcctactgactatatcatcaaatcggatggcctgaggattcttcaggtagattcaggctgccttcttgttgcagtcagtcatgcttattttacattcatatcatacagtgctgccatgattggagtcctcagcaatcagttattccagtcctctttgtttatactgaaacaagtcactataaaatctcctgttcacatggataaggtacagtatccagagaaagccaatcttctctagccttattgattttgtctcttagacttctccctgctgggaggcagaggttgcagtgagccgagatcacaccactttactccagcatgggcgacagagtgagactccatctgcatattccttgtgagagttaagctttggtcttcctcattttaccagatgggaaaccaaggccaggaagtttcagcattctcaccagctcttcagaaagctcatgtatcttggaagcagaatgcaggatggtgctggaggggcatatatttgtgagcccaggtaatttctgaatttctgatccaaatcttttcctccaaaatgcctgctaagaaactcagcagcattcttatgtttttactaaaacttctcctagaagagcatgttttgcttttaggagccagacttaagaaagtgcatcagcttaaaaatacatttgcttgtaatttttgtccatgctgccatctgacaggatttgaggatgcttccatttctgccaggataatagctttgttatctgctgagatctgcaatagctcgacagcacaggaaatctgtgtctcagccccctgctccaagtttagctcatccattacattccacaaactagtcagctttgcagcaacagcctcaccttcttggggaggcacatgatgtgagtcacacaattttcatgccagcccagagcgttgggtgccattacaaagccatgggtgtcttacatgaatgggagcctcgcggggggttgaagaggctgatctgatctgtggttcctcaattcagaggacatgagcttttgaaaataggcctttctaggtgaattggcctgcatgtcatagtttacacatactgagag

SEQ ID NO: 16169 - RNA, 1187 nt, Homo sapiens
  source 1..1187: mol_type = other RNA
gctgggattacaggcatgagccgtcatgcccggctttctttttgttcttcaagaaagggaaggaaaataacattgtctttgagccagttgcgtgtcgaggaaataagggtacccccccaccacaccccaaccccctcagtgccctggggtttgaagcaaatgctcagagggcctggtaggcggatgggcgtctccggatgatgcagaaagcaataagcaccagggcgaggaggccaagaaggatcaggccgatgatgagaggcagcaagatggaccggtcactggggcaggagaaactttgcccaaagacccctgtgtggggcagctgagcagcctggagcctcagggagagcaggtcgaggtggacagctggtgaaagaatgatgctcgagttgctgcaactgaagctctgccccaggggtgcttggagatctcgaagggatgcattctgagccgagaatgtccactgtgctgcgtgggggaaggacacattgtactccaccgccatgtagctcaggtagacaaccttctgctggaggtcctgcatgaatccaaagctgaggtgtccataggggaatgagagaagcaggtggggatgggcaccctcacagcttccctggaccttggttttgttggggttcagtacagagatgccccaggcctctcctccaccctgggttgtgtacatgactcgaatctgaatctgggcttggaggtggacacagggctgggaaccattggtccacgtgtagtctccaatggtctccttggaggttgggctaggactcggagagggtggaggtggttctgggtgggcagaactggtgaatcctgggctggtggcagtgctgttgcttgttggatgaaccgtggcatttccatgactagtggtggcaggactgtgagtggcagttgagggtccctggctggtggcagtgctattgcttgttggatgaactgtgacgtttccatggctggtggtggtggggttgtgagtggcagtcgtgggtccgtggctggtggtgcctgtggtggttgtcctgtgagtggtggttttgtggctcttggtagtcctgtggctggttgttccagtgctctctgccagtagccccagcagggcccccgagaaaagcacagccagcctcatggctgaaccgcctcacccaaagtccagctaggctgtctgc

SEQ ID NO: 16170 - RNA, 1268 nt, Homo sapiens
  source 1..1268: mol_type = other RNA
gctgggattacaggcatgagccgtcatgcccggctttctttttgttcttcaagaaagggaaggaaaataacattgtctttgagccagttgcgtgtcgaggaaataagggtacccccccaccacaccccaaccccctcagtgccctggggtttgaagcaaatgctcagagggcctggtaggcggatgggcgtctccggatgatgcagaaagcaataagcaccagggcgaggaggccaagaaggatcaggccgatgatgagaggcagcaagatggaccggtcactggggcaggagaaactttgcccaaagacccctgtgtggggcagctgagcagcctggagcctcagggagagcaggtcgaggtggacagctggtgaaagaatgatgctcgagttgctgcaactgaagctctgccccaggggtgcttggagatctcgaagggatgcattctgagccgagaatgtccactgtgctgcgtgggggaaggacacattgtactccaccgccatgtagctcaggtagacaaccttctgctggaggtcctgcatgaatccaaagctgaggtgtccataggggaatgagagaagcaggtggggatgggcaccctcacagcttccctggaccttggttttgttggggttcagtacagagatgccccaggcctctcctccaccctgggttgtgtacatgactcgaatctgaatctgggcttggaggtggacacagggctgggaaccattggtccacgtgtagtctccaatggtctccttggaggttgggctaggactcggagagggtggaggtggttctgggtgggcagaactggtgaatcctgggctggtggcagtgctgttgcttgttggatgaaccgtggcatttccatgactagtggtggcaggactgtgagtggcagttgagggtccctggctggtggcagtgctattgcttgttggatgaactgtgacgtttccatggctggtggtggtggggttgtgagtggcagtcgtgggtccgtggctggtggtgcctgtggtggttgtcctgtgagtggtggttttgtggctcttggtagtcctgtggctggttgttccagtgctctctgtaaccgtgggtgtcaccgtgaaggatggcagcaaagtagctgattttttgtgaggacagtcattccctgtcccctgggctgccagtagccccagcagggcccccgagaaaagcacagccagcctcatggctgaaccgcctcacccaaagtccagctaggctgtctgc

SEQ ID NO: 16171 - RNA, 1561 nt, Homo sapiens
  source 1..1561: mol_type = other RNA
gctgggattacaggcatgagccgtcgcacccagccaagtatttgtttcttaattaaggcagagtattctctctctaccttcagccttttcttcaaatgtgatggtttgtgctctgttcacttggctaagatggaactatcttttcgagatccctttccctgtacagttctgagttaaatttggccagaagaagaacttgtaccaggtttggaaaatgtgaagcagtggccatcactctcagaaagtcatcagggttagatgtggtgacagacacagagaggccagcgggttccagcttgtccttgctgtcctgcactccacatccagtcctcttcctgactgctgactccaggaccgacagcagccccagcccctccctcagatggcatttccacggaggagggaccacaggcttctcttttcagcccctccacagcagcaggatgtgcttagcttgtccaagggactgcttggcggctccttctctgatcctcccattcctccggggccttcacctctccagttcctcccaaagttgtgtaatgtccaattcctataataagtgtgtcctttatcccataactccaaggggttcccttccctgacttaaccctgactgttcagttaagaagtacttcccatgtctaaaataaatcaagacctcggaattaggacttccatttagatccaaagggatgtccatgggatgtaaagatgtgtaaacaccgtgaagacagctaaaagctcacccatcagtcttaccttccatgattatagggtaattgaaatatttgatttccccaagttctctactggcaaatacagtaccttcagccaaagcagtaaaagtcaccctttccttttcctcctgactttccttttaagcgagtgttcttgttcagaccacagtgtgcatatgtggtatgtatgtggtagcctgtcacttactgcaaagaagccctgagtccagcctgtaactgaatccattcctagaatcattaagcatagacaggtcacagaatggccccaccaaaatgcttcatgaaaggataggcattctttggcttgttgtacaattttttctctgccccaatgccatgggcagccgttcttttctgaccacccatgtgaataagctctggtaggatcctggattgtccctaccatagccttcatgatactgtgctgctattattcactggatgtctgtgtcatgcactagatggcaagtactcttaggacagtgtctctcatccagtcacttggcttcccggtgtccagcacagcacctgcagagtttggcatccggtagcaatgacttgaacccatggagtgtcaggtgaggagaggagaggccagcgctgtggtacaatggaaggaagggacaggaggcaaccacttggcttctcgccccagttctgccacttacaaaccatgtcacctgtgacaagtcaacatttgggagcctccacttcctcacctcgtgttctgcagcaggtggtggaagacaaacagctcagagctggactcagaacttggcagagtcctgctttcaactaca

SEQ ID NO: 16172 - RNA, 23 nt, Homo sapiens
  source 1..23: mol_type = other RNA
gctgggattacaggcatgagcct

SEQ ID NO: 16173 - RNA, 9160 nt, Homo sapiens
  source 1..9160: mol_type = other RNA
gctgggattacaggcatgagcctaccaggcccagcctcaagtaaaacctgataatactcaggcagaaagaaaatagtgtgaaaaaaccagtaatcagttattgctatattgtataggttgagagtctggaatggcacatatggtataatagcaatttaagaaaacatttatatttaccacttccaagcagaatcatttctgagtattctgcaaagttgatacaatctcttcatagagaagatgctctcttttagaagaaaagctttatgatgttatcagtaatactaaaaagaattataatctttgaaaacttgcttacttgtctgatttacttactacatataccaagccctagcttggtcctagtgtgatttttataaatgacagtgacaaacagtgtatctctaaaactgttgaatctttttttgttaacaggcacagttagaatacattgctatgttcatgagtagatccaaatatcatttagttttaaattttataattaaatataccatggattaatttgggtcatattacagtatagaattgtacatcactataggtccctaattttggacatgcatacttgataaataaatggctttttaaaaattgaaacatgctatagtctgttcaatttttaaacatgcaatatctatactaacatccctttggctggaaatgcaaggcatgcactgatgccaacttcgcttctggacatgcaatatctgtacttgtgcagacctatctgctgaatttctgcagcgtgtgcatgccacttcaaatgctacattttctttctgcactagcacagacctcattcacaaatatgcgacagtgactccatcactgatgagatgtctataatttgaggaattctgaactcaaaatctgatagcataaacacgacgatgttatacattcacaatttttctcgaatgaacaggaatgctttagaaatattaagttcatcattgagatgaaataaaaaggagagtgaattataagccagaaatgttttatgtggtttcataccaaagaatctataatcagctggtcaggggaggtataccctaaacatttttcttttagttaaaatggtcacatttgtttttgcagttttttcagtttctttcagaactaattaaaaagttaagttttcataaggttttaaagttgtcaagtaaatactctatgaaattagtgatggcctcacagaccacgaggttaaggagaggtgcatgtccacgtacaatgtctacgcaggaaaaatgagaacaatgcaattttcagatatattttccaggcttccacaactcctgagttaaagtggagaatttagttcttagcttcatgataaagttatcatagtatgctagcattatacatgacatcaaaatgacttaaatggcacaaacattttttacagaaagtcgttcaaggaggaattagaaaaaaaaggggaaaatgagagagaaaaagtattaaattccaatagctatacaggttacttaatatctgttactttatgtagtcctcacaacactgccattagctccaatttgtaaatgcagaatctgagatttataggaattaagcaatctgccccaattcacacagttaataaatggcagaacagggaattgagtccaggtttgtctgacttccaaacctatagtttcaacatttcactgtctctaaaaatatctcccaggataacacagaagtattttaaaaatcatattttattgttttttctaaaagactttataagaaacatgcatttggaaaatttccatggtatgagatgaaattaacaacaattacattttctcaattctaaggtgtcatcttttataagacactatattgattttattaataaaaaacattcttggtgggggaagaccctcacataaaatgtacttattgattttacaacacaattatttagaatcctaaaatgtgtgaaaagaatgtgtgtaagaatcaagggagatttttagctttattctccaatttgcaatttatggaccatatagatgttaacttacctctgaaagttaacatgaaattgagaggcttactatctgccctagtgaaatcataaatgaagttttatgttacttgagagtagattattaggatgagacagtggggcttaatttttgttttgttttaaatcaaatgtcaactggataaaataatgtttgaatgttatattgcctccaaagaaacagaaaacaattatatcaccaaagtgatttagaataacatatactagaattttaaaacaaattttaagaaatagatgtttcaaatcagagtgtttcaaatggctaaatttatgatcaccttgttattagttaaggacatgaatgattattcaggcagatgttaaaaataaatctttaccaatgagaaggatacaaaatagaagtttaaccattattatctctgggtgattctccttggttatttgtatttccagaattcactacaattagtatgtgctgcttttgtaataataattattcctgcttgttagcttttattttctccacttatttagagagagggttgaccagactggagtgcagtggaacagtcatagctcactgtggcctggaatttctgggctcaagcaatccttagccttagcctcctgagtagctagactacaggtacacatcaccatacctggctaattttaaaatttttttgtctagacaggggatctaaatatattgcccaagctggtcttgaactcctggcctcaagcaattctcctgcctcagcccccaaaagtgctgggattacaggcatgagctgcttgttagtcttaaaaaaaaaaagtgaattagatcgttttctatctgtctgttactaatctgtcttacaaatgctgtgttcatattatataaaaacaactgaaaaattcattggaaggaaaaaaattcaattttgtagactgaaaccaaaatcaatggactgaactggtttcattaacattacctatgttgtaagcaaatttttcagtatacaaacttggtaaatatagacaagaatttttgaaattggaattagacttgaaaatccaggacctgtggtcaccatatctatagaacttggaacacaggtgcatgataaacttttgttatgttacacacacttagctaagggttactgagtgctcagttctcttaaggaattacaactgttcgactcattcagggctaagaaagaactgaatctaaaaatgtccaggctatctaaaaaaaaaaaattataactgcacttacttctaaattcacttacacagaagacaggcaaagcagtcttccctgagctcatagaggcaatgcaggacagaagctacagttcccacagcgccagtgctgccctcaggagagctgtgcggccacatttctgactcctatcagtaacttgcaaagtagaactcttattggctcagactcacagtaattagaatagcaagactgacctgttaccattcagctattaacattaaagacaatcccagtatttccccaagcattctaggctgagaataatcaccactctgggataccattgtagtctcaattcccccttcccaaaaagttgcatcgtaatgtactgaagtgatgtcgtaagcaacagcactgaaagccagcaaaagcccacagggtttacttccatcagacgtccaatgatcatttatgaatcaatgaagtaggcctgcttcagaaacttgtagcaaacaatggctccatgggtaaagcgtaaggcaaagctgcttcattacatctactcagtgatgctcagccagagaaatgtctcatgagtcagtggagttcagcgggaatattctcgcaatgctggacgtcaaaaatagacagggcagcggatgcggctttctgattattacctgttgctttgagagctgcaatagcttgtggggaatttaggaaaagagagatcttgccattttccagaaatctcatttggattgcaaaacaaaaaagacagagaggcccaataagaatgacacagagcatgttgtctgcaatttaacacacaccactgtgttccaaaaatattcatttcctgtggcgacagcggcgaagaaacctcattatttttcgagcagcttgatcctgctttttggttagcaaactgctcctgagtttctgttgtacaatcacagccgtccggcgagcctgccgtcttttgccacatttcttataacttcggtagtacttttggatgagcacagcagcccgtcggctctgctggaattttttttgttcatagtaacttcggaatttgctctggataaggatggcagcctgtgtcatctttttataaagtgcgtacttcaaggctatccatgtcagctgtttatattttctgtaacaacgctgaataacagcagcagctacttcttgctgttcccgcaagggtcggcccttgtatttccggaaagctgtctggacaagcctggcagcctcatagagttctctctgttcatgatcagacagagtgagctgagcaaactcattctctaccttctcactggtagatgcactcaggaattctgaccaatccgcggcggagggaaggttaggtttctcgaaagcgatttcactgacgggagagccaacagggctcaagctggtattagaagaaggggttagaggctcgttatatgcacttcggatctgggcagcactgggaaggcagtcagcatccgctagataactggccagccagctcattgtactgctaatggtggcagggtctgttctttccaatcctgaggactccatgggcacaaaattctcctgcttgattcggtcaggtgtggcttcaataatgtgttctgccaaggtcatcatgttcacctgtatgtcatccatgggctggccgcattcttcattttctgcactatcacggtaggaccccagctctgtattcaccacctctctgttagccatcatcaggacactcattggttcccgtggacgcacctgtgaaggtgctgcctcctttcctacactggtccccttcggatttccagtcacctgtactgtagacacaccaatgtaaagatctttggaattccactttcctacaggctgagatccagaggcttgaaatgctgcagtctctggagtgggaggggagagttcccggctgaagtccctcactccttcactggggctgagtgtctcggggacagactgcttagaactagggctttgcttcctgatatttggctcttccagactcagtgcagtgggaagcagcttctcctgccttgtctggaagtactcagggttcaatttatgctttttgggagccggataatctttgtggctctcactgctgtagtaattagagggttcagaacgaggtcttctcagctctgggttggtgcttgcaataacagtgactcccttgggtatttctggagagctgatggcttcgctgtgccactgggccatccagctctctgtgctgggctcttcgcttgcaggacagtggattctggggttctgtcccagctgagcctgctcatctctctgcaggtgctccagacactctgctaatttcacatgaccccgtgacctggcaattcccaaaggcagccttcctagagagtcgggaatcgagatggcccgacggtcccacttgtacagcacgacggcagcttccaagtgccctagggcacacgcccacatcagaggagtacaggagaagtggtccacattcaaggggtcaacttccagttccaggtcaatgctatccgcgtgctttgtacgccatttgatgagggtctggattagggtggcatagccctgggcagcggccaggtggagtagggtcattccgcggaaagtctttgagtggatcaagtgcttggacttcgcccagcaggctcggctcatcatcttctcgcataccacgaccacacggctctcaaagcagctccccaaggccccagtcccagaagcacactgtgcctggctccctccattcccgctcccgctgccgcctccactgctgccgcctccgctcgcctgtttgtgctgctgggaccccgtcatctcggccatcctcctctccatctgctccagtcgttccaggatggacatcctgaactggttatcgtccaacgacagccagtcgtgctgggaggaagggagcgtgggcagagcccgggctttgtactcaaacaccaccgagttggagatgatctggttgttgaaggcaacttgtagggtcacaagaccagtgtcatgggctgggcagtagcagcgcagcaccccaggctgaatcagggatgcaggcactgagatctggtcaaacaggcagctgtagttattgctggcttcttgccacgggcctgtgatgaggaccttcactcctccctctgggtaagaccactctggggagtagtcggtcaccatgaacacccgtccgctctgctgcagcatgcctagggtgccctgggccgaggcggccgagaccacctcggcgacgtgcatgtaggccatggtgctggccccgccctccgagctgctcagctgcaggctaccctgctgggggctacagcaggggaggcacatctctgcctgggtgaagggggcccgcgccccgtcctctgactgtgagagcgccgtgctgtcccccgacaccagctggtgcccatagatggtgctgctgcccccctccacggagatgaagtcgttgatcaggtcggagaactggttgctgaaggagatgtcaaagtggtccaggctgagctccatgttggaggcgttgccgaggctgggctgggccacggggtagagtccctgcaccacgttgcccgggaggatggggacgccgccggcgcttcggattaccccgttggtctccggctgcaggtagtgctcagagctgcaagcctgcagctccccagacttgagcaggacctcgctcccttccgccgcctgcgaggtctccatggtgacctccccttctgccgtcatggcctggaagttggcctggaactgcatgaggtggagggaggaagtggactcgatccgcgtctccacgtgaccgctgcaggagctggtttgggacgaggcctccgttttcaccgtgggcatcacgaaggtgcccccagagtcactcaggctgctgtgggtgttctgctcgacggggaggggtttgctggcgtcctgcaggaagaagctcggggagggggtctggtggatgtgggggctgtggcccgtctggctgaagctggacgtgtagtccttgttggagtcgatggcgctgaagtccatctgctccagggtggtgctgggactcaggccgccgcccgacggcaggaggctggagccggcggtcagggtgagggagctggctgccacagccgccgcggaggaggagtacgcttctttggccatctgctgctcgaaggaggtgtcctcggtcttgatctccttggtgaggacggtggtaaagctgaagctccgctccccgggtggcgagtgccggatgttggagctgaccatctcggctttcaggcctccacccccgtacgtctggccctgctttgggttattaaggaaacagtcggggtcaaagttcatggtggtttctggaatcttccggccaccgtcgagggtggtggagaggaccagctcttcggacacgttggtgggcagcatggacaggctctccgagctgcccgtggtgggaaaggcgaacttgtggccatcagagctcacggccaggacgaggccctgagaggcgtcaggtgagaggaggtggtggttggggccagcggtgggggacatggtgtacacggcctcattggtgacctctgacatgaacaccgtggcgctctgggacaagctccccatcacagaggccaccgccataccggacacacctgtgaccaccgggctgtccaccatgtccgggtcgctgttgagcccgctgctgatggacacaggggagctctgggtggtgtcggggacttccacctggttggtggaggagacctcggtgctgctctggtgcaggagcacgggcttggccaccttgccgttcctcttctcacggctggagcccttgctgtggctgtgctcgtgcttgccctccgacacgtcattgtgctgcacctccgagtggctcccgtacccccctgtccgtggctccaccttgggcgagatgatgcggtgtttggcgctgttacacttgtgatgcacgctgccgccagctcccaggctgccggtgcagaggcagttgtgggtccgcggctggggcttggtctggtggctgtcgaggatctgctgcaccagctgttccaccgagaagcctgagctgctgttcccattgctgcaggtccacttgatgccatggaacatgggtttcagctgcccgatgagctcttctttcgtccatttcgcccactccttcttgtcggtgttgatggagcagaggatggggccgcaaggcttgccgcagtcctcgatggccggcacgttcaggtagtgcaccaggacgatgtcggggttctgaaggagccagtagcacctccggtggaaggtggggatgatggaggaatggacatagcagccgtacaagcactccactccctggaccttgagtttcatgtggtcctctctggtcgttttcccatctttcctctttttccagcaatacccatctttcctgtatttcactttcttcctgttgtagagtatcattgagccattctgtggtcttgtcttaggggaggtggttagccattcttcgtgtttctcaaatgttattaaataagctgcaatttcctcattagtgttccagcggtgcctctcttttggtaaacttgaacatttcggcagacattcaagcagctttttcggtaaaaagatttttacatgactactattgctgttcccatgatcatcttctataggtggcacggtgttgagaacacagtaggtgctagttccgcagaatacactttgggaaacgctcttccggcttgttttcggcagccatttcccctccgcgcgccacatcctcctcctcctcgcgaccgggaccccgagcgcgcgcctcgtaccgccgccgccgccggcccagccacccc

SEQ ID NO: 16174 - RNA, 1209 nt, Homo sapiens
  source 1..1209: mol_type = other RNA
gctgggattacaggcatgagcctcaaggtccagccaagaaacactttcaatccacaaagtcaaacttttgtggttctggtggctttattgtaagctaaattcattcaatagaagtgttaaaaaccagttcaacaaaagcaagtcctccatagctgtgagcaacgaaaaacacattctcagcagcagcctgagctatgaaatgatcccaaacatagattgcatgttcttcaggagaaccattttctctgatatacaattgcatcatttctttttctctttgggggttacgatacttctcatagaaatcacgtcgcttctttgtttctttagaaactttatcttttctttcccgtttttctgctggttcatctgaactatcagatgatgactgtacgtgtatcttcggcttttctacttcaatatagttttcattgggatttagtactattactccatatccttcagccacagctcttttaataaacggtatctgtgtgccactgtccagatcttcatttataataagtcttctagcccactgccctgccctgacaacaccactaccatgaattaaaaccatcagtttctgtggatttgtcaaagcatcctcactcataaagataaaactctttggttcactctcagtggcatctactggaatagatacttttttcaaattacaatccttttccaggagctcatatacatacttcgtgatgatctctcctagagcctcgtatcttttctggttccatctgtgtaaatcttcccggtagttaaaaacaaatggttccccagtttttatgtgtcttaactgtcccttttcattaaaagcatattcaaatccttccagggtatcaggaaaatcaagaggcggttcatcttttttcattagttcatccaaatctatcctagataataaatctttcagtgcggtagtcttttctttttcatctggacctccctgctggatttgtgccatgtttatccaaattggcaacaaaattaaagagctcaaggaaatagacatcaatcttcagaagacagtctgagctctgcccccagccacagggctgagggggcaggcgggaggaggcgtggccttccagttcgccagtcgaactccctcgtgcggttgttatgactttccctctcgggatccgcgccccgaccaagttcgagttgcacttccggggtcttcaggagatt

SEQ ID NO: 16175 - RNA, 2228 nt, Homo sapiens
  source 1..2228: mol_type = other RNA
gctgggattacaggcatgagcctccacacccagcccttccctgtatttctttaactcacacctgagcattgcataaactcagatttgtatttctgatttttgaaatcaattctaaattctggaagaagaattcaagccatctctgtaggatctaaatatcttgggagctgtaattttttttttctttagtaagttcccatcagagtcctgtagtattgctggtgtgctgcagaaaagccagcagatgccagggtctctgcctcatggtaagtggtttcccagggatgaaatgaaccttctgagtcacagacaaagtgaataaaacattttaagatatgcctgtgttggcaaactcagcagacctctggcgggaaggactcaattctctaacagatacagatcttaccagctgggaggcaagaggggagcaggtgaggcaggggggtgcatctgcagggaataccagccctccgccccaagggcagccccctgccaaagagaacattcaggtagttctcaatagagacctcataaaagcagctcacataaacaactctcgcttagtatctgtgtgtgtgttcactttaactgtctatgggttatttttgctgaaaagattctagtccagtggaaaatctcccctaacaaaaaaatttgaaactcttgttgaaccgtacagacttcccataggcaggcaggatcagccccattttccccaaaagaattgggcttgaaccctggagtcctgatcctgcagttgcactggtccgtgatgctgtgtccacaccctggcgggttcattccaggcttgataaccacatgactgtctgaggtcccagccttcaggatgcagcaggccccacgggctgaagggtatgtccatctgcattcaggtaggaggcaatggttttcctgaaggatcagtgctcagggtggcaagtttcccaacgcttcccagtaagcaacgcactatataaagacttcagtttaagtcacaaactaatgtccctgcatctcctgtaggtgacattttgagtggtcattaaagaaatgtatctttcaagaaaacaagctgctcaatgcttagaaacgtgcattgcacctatcagtctttttgtgatcctgttataggtatcctggttctatctagatctaacgggataatttttgaggacggggacaatattttcatatttcagtatctttcatagaattgcttctactttcagtttctatgaagctaatagttaaacatgaaaagttctataatgaatagctttatcttctttaaaacaaatttagtaatttcatgcatgtaattttattaatccacaatagcaaagcaggaaaagaagtacaaataaaagaaaagctcttttattttagacatgtccgtgatggcagcataagtttcagtgcatgtagaccaggggcccagtacgctgctctggaactggacttgggacacagcagctggtgatgttctctcaagagcaaataggcgcagccattctcctgcttggctgactccttcccactgcttgccagtgatgcttgtagtcgcacatgcgggacagggcaatcatcatggcgcagtacaagggcaggatggcagcacagagccgccagctctttccccgcccactctcggtgaagcagtgcagcttgcccgccaagtagaacgtcgtgaagccaaggcccgaaaaggcaaaaacatgaggcgggtaggtatgttatctgattgcaccaaaggatttttatagagccagatctcttctggctggatgactctctggaacggatccaaaaactctgtaaaaacgaagactccgaagagcagggctcgcaccccgatctcaatggccagctcccgcatggtgcggccggagcagctcccgcggcgtcagctggtgctctccgcggctcccgcagctcggccggcgccggctcgccagaccctgggaggcgagggaggcgcgctccaggccgcgggcgggggcggaggcgggcgccgggcgggggcaggcgccggggagggctcagcctaaacctcgcgcctcgggctccggggctccgggaagccgcgccggccgctggcgatactgcggaccccgcctcctagtgcggagccggggccgcctcagggactcccggatccctctccccaggagccgcctccgcctcctgggcccgcgccgggcacccgcggaccggggaggggaagcccg

SEQ ID NO: 16176 - RNA, 2508 nt, Homo sapiens
  source 1..2508: mol_type = other RNA
gctgggattacaggcatgagcctccacacccagcccttccctgtatttctttaactcacacctgagcattgcataaactcagatttgtatttctgatttttgaaatcaattctaaattctggaagaagaattcaagccatctctgtaggatctaaatatcttgggagctgtaattttttttttctttagtaagttcccatcagagtcctgtagtattgctggtgtgctgcagaaaagccagcagatgccagggtctctgcctcatggtaagtggtttcccagggatgaaatgaaccttctgagtcacagacaaagtgaataaaacattttaagatatgcctgtgttggcaaactcagcagacctctggcgggaaggactcaattctctaacagatacagatcttaccagctgggaggcaagaggggagcaggtgaggcaggggggtgcatctgcagggaataccagccctccgccccaagggcagccccctgccaaagagaacattcaggtagttctcaatagagacctcataaaagcagctcacataaacaactctcgcttagtatctgtgtgtgtgttcactttaactgtctatgggttatttttgctgaaaagattctagtccagtggaaaatctcccctaacaaaaaaatttgaaactcttgttgaaccgtacagacttcccataggcaggcaggatcagccccattttccccaaaagaattgggcttgaaccctggagtcctgatcctgcagttgcactggtccgtgatgctgtgtccacaccctggcgggttcattccaggcttgataaccacatgactgtctgaggtcccagccttcaggatgcagcaggccccacgggctgaagggtatgtccatctgcattcaggtaggaggcaatggttttcctgaaggatcagtgctcagggtggcaagtttcccaacgcttcccagtaagcaacgcactatataaagacttcagtttaagtcacaaactaatgtccctgcatctcctgtaggtgacattttgagtggtcattaaagaaatgtatctttcaagaaaacaagctgctcaatgcttagaaacgtgcattgcacctatcagtctttttgtgatcctgttataggtatcctggttctatctagatctaacgggataatttttgaggacggggacaatattttcatatttcagtatctttcatagaattgcttctactttcagtttctatgaagctaatagttaaacatgaaaagttctataatgaatagctttatcttctttaaaacaaatttagtaatttcatgcatgtaattttattaatccacaatagcaaagcaggaaaagaagtacaaataaaagaaaagctcttttattttagacatgtccgtgatggcagcataagtttcagtgcatgtagaccaggggcccagtacgctgctctggaactggacttgggacacagcagctggtgatgttctctcaagagcaaataggcgcagccattctcctgcttggctgactccttcccactgcttgccagtgatgcttgtagtcgcacatgcgggacagggcaatcatcatggcgcagtacaagggcaggatggcagcacagagccgccagctctttccccgcccactctcggtgaagcagtgcagcttgcccgccaagtagaacgtcgtgaagccaaggcccgaaaaggcaaaggaggaatggatgctggggaagcttttgcggccctcggacaccagatcggggtcacctgtgcaatgcatttccgagttcatcactccatctggaaagcagcggtaaaagaaatcggggcgaggtcttcccactattaatttaatagtgtttgtgcagactccattcaaagcaagagccaaggacaccgctaagaaggcttccttaatttcagtcttgtctgttcgccggataattttcaccacacaaataacagccaggggtgtgaggaaagaaattgcaaacatgaggcgggtaggtatgttatctgattgcaccaaaggatttttatagagccagatctcttctggctggatgactctctggaacggatccaaaaactctgtaaaaacgaagactccgaagagcagggctcgcaccccgatctcaatggccagctcccgcatggtgcggccggagcagctcccgcggcgtcagctggtgctctccgcggctcccgcagctcggccggcgccggctcgccagaccctgggaggcgagggaggcgcgctccaggccgcgggcgggggcggaggcgggcgccgggcgggggcaggcgccggggagggctcagcctaaacctcgcgcctcgggctccggggctccgggaagccgcgccggccgctggcgatactgcggaccccgcctcctagtgcggagccggggccgcctcagggactcccggatccctctccccaggagccgcctccgcctcctgggcccgcgccgggcacccgcggaccggggaggggaagcccg

SEQ ID NO: 16177 - RNA, 4845 nt, Homo sapiens
  source 1..4845: mol_type = other RNA
gctgggattacaggcatgagcctccacgcccggcgtcattgaacttttttattcaaaggggtagaatgtatatgtgggacaaagaaagaggctagattaacaaagctatcatttccttgtttctctttgacagctggtcaaataattcaggcatagctaggactgatgctcaagttagaaacaggtggcccatgctgtccaatatagcagccactagccacatgtgcttatcaagcatttgcactgtgtcccatgcaacaaggaactggattttaattttaataaatttaatataaatttttaaactgatacttatttcaattcttgaaaaaaacttttgtcttagctacttgatatgagaatctgttttcaactgtaagttgtatgaaatctaaatacagatcaagtatgtccaatgaacattagcatccaaatggagatgtgcagaaagtgtaaaatacacaccagatttcgaaagcttagtatgaaaaagagaatgtaaaatgtctcactaatatatttttatatgttgaaatatttggcaaatgttggattaaataaacttttattaacattttcacctgcttctttttatgtttttaaaagttgctactagaacatttaaagtgacctatgttgttcatgttatagttctcttagtgtagaggtagactgttatagagccagtgaaacttgacttataaatagctatgtaaccgtattttctgaataatcacctagctatccagagtgagtaaacactcacttacttaaatatttaatttcctggagaaaatgtggattggtgggctttgaaaagttggtaaaaactttgtgttttaagaataaaattaaacagtttaaacgagaacctgaaataatacttagggcttaacagtgtttgtaaaaaattgttatctttgctctagtcaggcctgatttaacattagtttggttgatacatataagatatatatcattttggaagttttgtgaattacatataataaaatatagcttagcaaatatgcaaccaaaatgtttttatcttctctcaaacctgaagaattctctattactctaacctccaaataacttatttgatttagggagaaatcaaggatgtctaaaacaaaacaattgatggaaaggctctattaattttagagtagattaccccctactccccatcagcattgttaatttagatatactagtgcccaccttcttttctcaaaaatcccctaccagcttacatgaaagtggtaaaagaattcaataagcttagcttgaaaacctaacccaaacataatttaatcttttgatgatgatttaaaaatcatacaattacagacacatgctggctacaaagtctctgaggctcaaagttttaagattagatgaagattagctgggtgtggtggtacatccctgtagtcccagctactagggaggctaaggtgggagggttgcttgagcccaggaattcgaggttacagtgagcaatgattgtgccactacactctggcctgggtgatacagtgagaccctgtctctaaaaaaggaaagattaggagaagatattcactttgtgggatttaactagtctgcaataaaaatgaattataagcttccatctccagaaagttatcagacacaacacgtagatcaacattttcaggagatcagttagaattcagtagagtatatataagacttaaattacactgaataaagttttatgttccagaatagtgaagaaagctttaccttcatgaaaatcaaatctcttttctgacaaaaattcagaatttagggtgaatgtcttgatccaattttgtattttaaacttaattaaaattttgatagccttctgttgaaaaatatgtaaatttatgtttctcagaaaagacgaattcagaattttaagaaatcctatgcttttggctatcttgttacatgaattttgagttaaaatactgagtttatgagtttgaatctttctgaagtgttaacacaataagcccactgtactgcataaagataaaacgttgagggttactttgtcttaggggactggaaattattaaaagggcaaattccccatacattgtgatctgtcatatttagccctgacttgtcttgtggtaacaactgtgttgcctaagaaaaataagaaaatagaacaaaccattctgcccagttcaaccaaaatgactccctttgtcctagaaaacaaaaaaacataactggggaggttggcaagaccataacctatggctgtgaacatttaaaccttacagaaaaactgagatcaatgcccccaaagaaaaactacccgagtctttatgagacattgcagattaaaatgaaaaccattcaataatattgaaatgctcaatacaaatcagtaccttagacaagacatacacacatcttgctacctggatggagggcattataaacatcagttagccatcacagctctcacagaagcatctgcaagtcaatggtgtggagagcctgatttcaagcgttcaaaatccagtcagagctggcttataagaagagcccaatcaagcagtcaaacgtgtttacaggtcagctctgctcctggccaagtggcgttggctggggcacgtggtgagtgggtggtggcggaccaggctcctgtgtcagctgcaggtgctgagctggatctgaagtacttgtagctaaatggagctcctctgtttgctcttgatgggcatgaagatgttccagtgtttccttggacagagtgatcacgtgcactggctctgtttgtgagggccccatctggctttcaatcatattgaggctctgaatgtgttctgtttgctcctgttgagctgaaagaattaaattctgcagttgctctggctgctgcgtgagcagggtaagattagcagcctggtctgcagtcatgttttgggaactctctgcagtcacaatgctgattccctggctaggaccgggcatgaaattgatgttatgtacagaatcggttacgagaagctgaatttcctgctctcccgaggtagagagttgatatggctgtagctgaagaatattcctgacctcttctgtattactactgccagaaatgctgctggcatctgaagcatgcttctccttgctatgaattttcaagtgagccttcaagttgtctaagcgagcaaactgtaagttacactcagggcaggagaaaggcttcttgccagtgtgtagaatgcagtgtctccttttggcactggagtcagagaaggatttgccacaaatgccacaggagtatggcttttctcctcgatggattctgatgtgggtctgaagagaactctttgctgtgaaagatttgccacagatttcacaagtaaatggcttctcacctgtgtgtgttcgcagatgtttctttagctgagacacatccatgaatttgcgatggcagtctttgcattccggtaatgagtggcctgtatgaactcggtaatggctctttagctgtctgttctggctgaaatattttccgcattgatcacaggtaaaagacttctgtcctgagtgcaggctcatgtgctccagcagtgagtgcttggtggtcagagccttgctgcacacggtgcaggtgtacggccgctcgcctgtgtgcatcctggtgtggacctgtagcgagtgcttctgggcaaagccttttccacactcattacatttgaaaggtcgctcccctgtgtggctcctctggtggattgctaaaaagtgattgtacttaaagaccttgccacagtctttacagcgggcctcagggcctccagggcgctttctccttccacagatcctcttggctgaaccatggtcctcttgatccccaacaagtttgtaatctttaagtttgacggatctccaaatcctccgcttgctgtatcgactctggcttgcctggccatcctcggtcttgggatcatagttctcatctttttcaactggcatttcctcctctctacttggctcacaagtaggctccgattcttccttttcttttgctgcaatttgctcattcagtacaccactgtctcctttaaccacaaagttttgtctattctgaactgaattgttcactcttaactgtatttcttcctctgcagccagttctgatttctcctcctgcaatgtattgactttttttggtcttccccgtttccgctttggaggatcgtttttcttattagagataacaaccactggggcaccagcagtgttcaaagttgttggctttggggagctatgattattttggaagtctgtgtaagcctttaccaggtcatagacttttaagaactgagcagtagccaggatttgttctgtacttttctcactggcatggagataacctgtgtagataaattccagcaggataccaaaggtgtctgcaaccatgccttccagcatataaatggattggccgatttccccctcttctgcaaacatcattgagaagtattcactactggcagcaagtaaggctttgtgggcccggaaatgtacattctccacgattaaagtaatgtcacagaggaagcctttcttcctctgatcctcaaaactggccagcacagtgtcactgtgagcgtctgagtgtacaacaagctgcccagaaggctctggcgatgtttctgccattttcttcagaagccactaagggttaaatccggcggcctggcgggagacccacgccggggcccgctggccctccgctccgccccgcccgcctctggggcttctgcgccgcaccggtttctgctcctgcgccgccgccgcagccacagccac

SEQ ID NO: 16178 - RNA, 1518 nt, Homo sapiens
  source 1..1518: mol_type = other RNA
gctgggattacaggcatgagcctccatgcccagccaaaagataatcttttcaaaaatggtgttgaaacaactggttacttatatatagaaaagaaataactggttatgtatatagaaaagaatgaaccataatccctccctcaaaccatatatgaacattaaacagatcatataccaaaacagtaaagctaaactaaaagctactagaaaaaatatgcaacttttgggtatacaaaaattttgtaggtagtacacacacaaaaagcacaaaccaccaaagaaaataatttacaaagtaggctttataaaaattagaaacctctgctttttgaaagacatagataagaaaatgaaaaggcaaaccacaaacctggagaaaatattcataacatatatattagacaaaagttgtatttccatattatataaataattctaaaaattcaataatagggagacaatcaacctaattgttttttaaaatggttaactgatacaaacagaccctacataaaagaacttatatgcatagccaatcagcatgtgaaaagatgttcaacgtcattagtcatcaaggaactagaaattataagcaaaatgggataccattagagacccactaacattaaagaaactgacaatttcaagtgttggaaacaatgtagaacaactgcaacaaccgtaaatttctggtggaaatgtaaaatggcaaaactactttggggaaaaaatggctttttttagaaagttgaacgtatactcctagggatttatataagagcttgaaaaacatatatcaacacaaaggcctatgtatttatgcttaccccaactttatccaaattaatctaaagctaaaattaagacaaatatccatcaatagatgatggacaaaacaattgtgatatatctatataatggaataggatttagcaatctatataatggagtataattatatgaatgtgatacatctatataatggaataggacttagcatgcattcatccatgcaccaacatggatgaatctgaaaagtgtttagattagcaaaagaagatagatacaaaataagttcatattgtataattccatttatataaaactgcacaataagagaactaatgtaaagtgagagaatagtgattgcttggggctgagatgaaggatttgtatcaaaagggcagagaagagcttgttagggtaattgaaacgttctgtatcatgatgtggaggtgtttacatgggtgtataagcttttgagaacttatcaaattatacacaaatatgtacattttattatatggaaattatatctcattaaagttgatacaaaacaagaatccagaactctattttgacatctggtggacatcgctccaatcatgattccatgtctctcgtgtaagatatccatggattttctttttccagaaactttataggccaggaaggagctggatgatatattcaaaatcagtttcacatggctgcggaagcctcatggtcatggtggaa

SEQ ID NO: 16179 - RNA, 2271 nt, Homo sapiens
  source 1..2271: mol_type = other RNA
gctgggattacaggcatgagcctccgtgcccggtgcatccctaatcttgagcatgatctcagtcggcaaatgaggccatctgttttcagcctgtttgaaaataagatgtggggaggccatgatggaaatagcacgtggggttaaacataactggcagatgtgggagcgatggtggggcatgccattcaaacaggtcccaaaatgggtgcaacaaggtatagcacatctaccactcgctaacttgactgacttggagaaatgactacacttttgcctgtttcctcagttggaaaatagccatattaacacctctttcattggcttgctgtcagggtactgggatggggggaggtgcatgggttggggtggccaccaggtggtgctgtgccacagcgggcagcccctctggaaatgactggcatcataaaatctgtcttcatacccgaggtagtgttttttgtttttttaagatctctaccttttaaaagcgtggcatacagtgtgcttggtattgtgttaggcatttagacgtgctcaggttgtaaggttgaagtgccagtctttgaatattctgtaaggattgtgagggtgtgaggtggttttgagtctggtcacgggtcttgtttcctccgggagagggtgggtacaccagccctcaggcccaggtgcggcactgtgggcggctttcagcctttcccgttctgtaagcattgcagattcccaaggaaaagcgagcctttaccatgtgggttttctttgttcccagcacatcgtccagagtttcatcccagctcctaggagacaggccttgcaggggtgtgtccagccttgtctagagaaggccgcctttcatgcagtgcttcccagccctggcttgtgactcagtcatctggggcacttaggcagttcactgtggtggccagggctgactggagattgcgattgcggtggtctggggcataggtgtgtttccaagctctcaggtgggcctctgctttgctggggcttcagcaagcccttaagtgctgcataccaggtgaatggggaggggggaggtgatgggctacagctgctggtgtgccgactgtcctccaactccctgctgagtctgtgggaggtctgtctgttgtgcttcagctttttgacacctctctgggtcagcaggcctccggggaagcagctagaatggtcgctgtctggctgggtgcaggtgggctgacaggtttggatattccaggccgcattccggtggctgtggagatagccctgagggacagcctttgcagtttgtttcttccagtgccgtgtgcaggcctccagccttctggggctcccttgccccgggttcaaagtcagtcctcggtgaccacccactgcctaggaggcaggcccttcccacctggggggcctctgagggcaggggctgtaaaagcagctaccagaagagtccactttccccagcaactgcagggaccctgactcctgcttgtcctgcagcctgggctcctccctccgctggccaagtcacgccaagcagtttgcggttacaggacgggtgggggcctctgcatatgtgcagagtacggagggcccagggacgcgaggctccccgatgggcaacctcccctgcctttgcttttccccagagccccctcctggcctgcgttcggcatcttctcgggtcgtcatcgccctctgcggtgcctgcgctcggggtgagggtttttgtcggcttttgttacatcaccgatgtaacagtgcctggacgtagtaggtgctcaataaatatgttgttgaatgcgcttcagtctccccgaatgcttgtcccttccgggcgctctcatcgctctcctaccttccccgctacacagctcgaaggtcccctcctccgggaagctcaccctgtcccacttgccaggaagaatcaagcaaattttctgagtgagacaccttgtcctcactcaggcgtcctgcaggcggcttcagcgagttgttggggcagatgcgccgggagctcccgagggcagggacggcgtcttatttctctttttaagtccacagggcttgcacaatagatgcccaaaaaatgagagtgaatttagaatgagtgaccgagtggctgaagattgcctccttcctttcccagtctgtcggttacttaccctgtgacaagcccttgggacgggcagtcgcccctctctggcctatgactgctggctgcccccactgacaccttatacccttgatctgatcataaataagaagcagccc

SEQ ID NO: 16180 - RNA, 1486 nt, Homo sapiens
  source 1..1486: mol_type = other RNA
gctgggattacaggcatgagcctctgcacccagctgacttcttcctttattatttatttattttgagacggagtttcactcttgttgcccaggctggagtgcagtggcgcgatctcggctcaccacaacttccgcctcctggcttcaagagattctcctgccttgggccgagcacggtggctcacgcccgtaatcccagcactttgggaagccgaggcgggtggatcacctgacgtcaggagtacaagaccagcctggccaacgtggtgaaacccatctctattaaaaatacaaaaattagccgggcatggtggcggatgcctgtaatcccagctactcgagaggctgaggcaggagaattgcttgaacccgggaagcgggggttgccgtgagccgagatcgtgccattgcattccagcctgggcaacaagagtgaaactccgtctcaaaaaaaaaaaaaaaaaaaaaaaagagattctcctacctcagcttcccgagtagctgggattacaggcatgcaccaccacaatgcccggctaattttgtatttttagtagagacggggtttctccatggtggtcaggctggtctcgaactcctgacttcaggtgatccacccatcttggcctcccaaagtgctgggattacaggcatgagccaccgcgcctggctgacttcctcttttattacttatcttcttgaccctgccttggctgttgggctctaagagcatacaaattctaccacctccagctaccaatgcgagccaagttctgagccttgagtgggaatgtggcacaactgggcactgggtaattaagtcctgggtccaggccaaaggaggacccagccttatatggagttcataggacagaggcacatgactttcttaggaggcagccaaaggcctctggactgatcagggcatcggtggcagaggagcagggtgacaggccgcctttggctgggctttatctgggctgatgctgaagctgtagaggccctggagcacaccattcaccaccacgttgggcagcgactctggggaggggttgcaaacatagggatccacatggaagctcaggacaggccgctggtgctgctgggagctgctgtcgccaggcaggaactccctcagggtgccccagttgctagccttggggtctgtggggaagtgccgaagtctcaggaattccagtaactccttgggcacctcctggttcaggtacaggatgccctggatgtaagcctccaagccctgccggcgctgttccaaccctctggtcctccagttgggcaggcgtttcgaggggaagtcgggcactttgtacagcttcttgatcatgtggcttttctccgggctctgcctgggcccctcggcctcgggccccaccgacgggatgtgaacttccagcatccgcgccccggccccagctgctccgcgcgctcggctcggagccctaactctcccggagcggactgagga

SEQ ID NO: 16181 - RNA, 1546 nt, Homo sapiens
  source 1..1546: mol_type = other RNA
gctgggattacaggcatgagcctctgcacccagctgacttcttcctttattatttatttattttgagacggagtttcactcttgttgcccaggctggagtgcagtggcgcgatctcggctcaccacaacttccgcctcctggcttcaagagattctcctgccttgggccgagcacggtggctcacgcccgtaatcccagcactttgggaagccgaggcgggtggatcacctgacgtcaggagtacaagaccagcctggccaacgtggtgaaacccatctctattaaaaatacaaaaattagccgggcatggtggcggatgcctgtaatcccagctactcgagaggctgaggcaggagaattgcttgaacccgggaagcgggggttgccgtgagccgagatcgtgccattgcattccagcctgggcaacaagagtgaaactccgtctcaaaaaaaaaaaaaaaaaaaaaaaagagattctcctacctcagcttcccgagtagctgggattacaggcatgcaccaccacaatgcccggctaattttgtatttttagtagagacggggtttctccatggtggtcaggctggtctcgaactcctgacttcaggtgatccacccatcttggcctcccaaagtgctgggattacaggcatgagccaccgcgcctggctgacttcctcttttattacttatcttcttgaccctgccttggctgttgggctctaagagcatacaaattctaccacctccagctaccaatgcgagccaagttctgagccttgagtgggaatgtggcacaactgggcactgggtaattaagtcctgggtccaggccaaaggaggacccagccttatatggagttcataggacagaggcacatgactttcttaggaggcagccaaaggcctctggactgatcagggcatcggtggcagaggagcagggtgacaggccgcctttggctgggctttatctgggctgatgctgaagctgtagaggccctggagcacaccattcaccaccacgttgggcagcgactctggggaggggttgcaaacatagggatccacatggaagctcaggacaggccgctggtgctgctgggagctgctgtcgccaggcaggaactccctcagggtgccccagttgctagccttggggtctgtggggaagtgccgaagtctcaggaattccagtaactccttgggcacctcctggttcaggtacaggatgccctggatgtaagcctccaagccctgccggcgctgttccaaccctctggtcctccagttgggcaggcgtttcgaggggaagtcgggcactttgtacagcttcttgatccgcttgtgcagcgcgtggaactcgctgtagcgccttggcaccgtgtgtctgcgcccgctgcacagcacctccactcggaacaccatgtggcttttctccgggctctgcctgggcccctcggcctcgggccccaccgacgggatgtgaacttccagcatccgcgccccggccccagctgctccgcgcgctcggctcggagccct

SEQ ID NO: 16182 - RNA, 1593 nt, Homo sapiens
  source 1..1593: mol_type = other RNA
gctgggattacaggcatgagcctctgcacccagctgacttcttcctttattatttatttattttgagacggagtttcactcttgttgcccaggctggagtgcagtggcgcgatctcggctcaccacaacttccgcctcctggcttcaagagattctcctgccttgggccgagcacggtggctcacgcccgtaatcccagcactttgggaagccgaggcgggtggatcacctgacgtcaggagtacaagaccagcctggccaacgtggtgaaacccatctctattaaaaatacaaaaattagccgggcatggtggcggatgcctgtaatcccagctactcgagaggctgaggcaggagaattgcttgaacccgggaagcgggggttgccgtgagccgagatcgtgccattgcattccagcctgggcaacaagagtgaaactccgtctcaaaaaaaaaaaaaaaaaaaaaaaagagattctcctacctcagcttcccgagtagctgggattacaggcatgcaccaccacaatgcccggctaattttgtatttttagtagagacggggtttctccatggtggtcaggctggtctcgaactcctgacttcaggtgatccacccatcttggcctcccaaagtgctgggattacaggcatgagccaccgcgcctggctgacttcctcttttattacttatcttcttgaccctgccttggctgttgggctctaagagcatacaaattctaccacctccagctaccaatgcgagccaagttctgagccttgagtgggaatgtggcacaactgggcactgggtaattaagtcctgggtccaggccaaaggaggacccagccttatatggagttcataggacagaggcacatgactttcttaggaggcagccaaaggcctctggactgatcagggcatcggtggcagaggagcagggtgacaggccgcctttggctgggctttatctgggctgatgctgaagctgtagaggccctggagcacaccattcaccaccacgttgggcagcgactctggggaggggttgcaaacatagggatccacatggaagctcaggacaggccgctggtgctgctgggagctgctgtcgccaggcaggaactccctcagggtgctgctcactgctgacagcccctggcccccgccatcggccccccttacccccagttgctagccttggggtctgtggggaagtgccgaagtctcaggaattccagtaactccttgggcacctcctggttcaggtacaggatgccctggatgtaagcctccaagccctgccggcgctgttccaaccctctggtcctccagttgggcaggcgtttcgaggggaagtcgggcactttgtacagcttcttgatccgcttgtgcagcgcgtggaactcgctgtagcgccttggcaccgtgtgtctgcgcccgctgcacagcacctccactcggaacaccatgtggcttttctccgggctctgcctgggcccctcggcctcgggccccaccgacgggatgtgaacttccagcatccgcgccccggccccagctgctccgcgcgctcggctcggagccct

SEQ ID NO: 16183 - RNA, 1305 nt, Homo sapiens
  source 1..1305: mol_type = other RNA
gctgggattacaggcatgagcctctgcacctggcctggagacaggtcctttcatcagatgattaacttaaatgagaccttcagtgtgggcccaaattcacatgactggggtccataaacgaggaggacatttggaggcagagagaccccacgagtgcaggtgcacagaggaaaggccagagaggacagggccggaagggaccccctgccagccaggaggagcgactgcagaagacacaaccccgcccacccctccaccttggacttgcagcctccagatgtgtgagaaaataaatgcctgccctgtgggcacccagcccggccatcttctatggcagccgaagcctgaagctctgtttccatggaggcagctccttctcaggggctcaggttggcctttaaggatgttgctcaaagcttctgactgccgggcttgtgactattcatgcccacttactacgtccagttttacgacaaattcggttatgccagggagatggaaggggccaggttggggctcccaggctgtgggggtggatggaggttgctctggaggcagaaggggcctctcactcacaggaagggcccaggaaagcaggtgggaggcagggaggtggagggagcacgaggagtgtgggtgagggagtgtaaccacgagggcaggcagggggcaggagggaaggcaggagggcctggccaggagaggacctggtctggaacagaggggaggcctcaagaggatgagcaggaggtgagaggagcgaggcgatgagcctggagggagaccctcacctgagaatctcccccagcatgatgtgcagtaatatataatatttaggcagattattccaaggctcaaatagctctctttggctgtacacgaacttgctccaacagtgctgaaattcgtcataattcatgatcttcatggtggcacgcggaccgtctcttttctgacacaggctgcgaagcgcctcctggtaatctgggtcccagaagtagtagaggcgggcaacaaagatggtcagggtaaccttcgggtcctcggccaggaacgtggccatatcccttgtacactttgtgcaggggctccaggatatgtaccaggtgacctcatactcctggtcacgatgcagcttcctccacttgctgaaccagtggaagaatctcatctctgggtggtacttaagttcggaatacacctgaagtgaggcttcatccttggccggctagtcccgactaagatctttgtctggagcaccagggtttcactttctgctccaagcttctggttttaggacagccc

SEQ ID NO: 16184 - RNA, 1459 nt, Homo sapiens
  source 1..1459: mol_type = other RNA
gctgggattacaggcatgagcctctgcacctggcctggagacaggtcctttcatcagatgattaacttaaatgagaccttcagtgtgggcccaaattcacatgactggggtccataaacgaggaggacatttggaggcagagagaccccacgagtgcaggtgcacagaggaaaggccagagaggacagggccggaagggaccccctgccagccaggaggagcgactgcagaagacacaaccccgcccacccctccaccttggacttgcagcctccagatgtgtgagaaaataaatgcctgccctgtgggcacccagcccggccatcttctatggcagccgaagcctgaagctctgtttccatggaggcagctccttctcaggggctcaggttggcctttaaggatgttgctcaaagcttctgactgccgggcttgtgactattcatgcccacttactacgtccagttttacgacaaattcggttatgccagggagatggaaggggccaggttggggctcccaggctgtgggggtggatggaggttgctctggaggcagaaggggcctctcactcacaggaagggcccaggaaagcaggtgggaggcagggaggtggagggagcacgaggagtgtgggtgagggagtgtaaccacgagggcaggcagggggcaggagggaaggcaggagggcctggccaggagaggacctggtctggaacagaggggaggcctcaagaggatgagcaggaggtgagaggagcgaggcgatgagcctggagggagaccctcacctgagaatctcccccagcatgatgtgcagtaatatataatatttaggcagattattccaaggctcaaatagctctctttggctgtacacgaacttgctccaacagtgctgaaattcgtcataattcatgatcttcatggtggcacgcggaccgtctcttttctgacacaggctgcgaagcgcctcctggtaatctgggtcccagaagtagtagaggcgggcaacaaagatggtcagggtaaccttcgggtcctcggccaggaacgtggccatatcccttgtacactttgtgcaggggctccaggatatgtaccaggtgacctcatactcctggtcacgatgcagcttcctccacttgctgaaccagtggaagaatctcatctctgggtggtacttaagttcggaatacacctggcctcgaaagatctttgcgtccaaagggggccttgagggaccctttgttttcacttcgtagcacagccagacggtattccgacgagaaaggatgggtctattataaaagttgtaggagaatgtgtctcgatacattcgctccactgtgtttctgaagtgaggcttcatccttggccggctagtcccgactaagatctttgtctggagcaccagggtttcactttctgctccaagcttctggttttaggacagccc

SEQ ID NO: 16185 - RNA, 1513 nt, Homo sapiens
  source 1..1513: mol_type = other RNA
gctgggattacaggcatgagcctctgcacttgggcccacttcttcaattcttcttgccatttcttgaaccatatttccaaagtctttttctggttatttatgagacacaacttgatgctcagttaaaataagtgaggtccgctaacactcagtagtgcagctgaaacctattcacattcaagtcacgaaatagaacttgtatgcccttcagctagaggaagtggggctacctgacataaaggtagaaaaatcccctgacactcggaggagataaagtgtcatgacttagatagggcatataggagataggaggtttcatgactctcaggtaagggagatgagacctccagacaaccaggaagaggtgagaatacctccagacctcagggggttgagatgagaactttggacacccagaatagaggagatctcatgatactctagcagaggagatgaaagctccatgccatttagacagggatatgagactatattcaagtagagggtaggacatgccctggcacccagatgggggcaatgagatctcccaacactctggtataccggtggagacttcagaacattcatataggtaaaatacaacctcttgacattcagctggaagatgtaagacctcttgattttcaggtagagaaagtgcgacagggtgacacttgggtggtggaggtgagaattcttaacctgtaggtggaggcgatgagggcctctggcaattcaggtagaagaggtaaggctgccctcatgcaggtaagagtgtgacctcctgacacttgcaggcgatgggaaatgttttaacattcaggtgtttgcaataagcatttgtcacactctggtaggtgagatgctagttcctgatgatcagatgggaaaaatgatgcttcatgatattcaggtagctgtatgaaaactcttgacattcaagtataggagaaaacaccttgctccacctcagtcacagaaagccgatctggagacattcaggataataggagaccttgtgatattcagcaacggacaggaaggtgggctttgcagttgtaaattaggaaaattcaaaatgactcttggaaaagtgtgttgatagcattcacttggaagaggaaaagaaaacttccccaacaacaattaaggatcaattaatctgctgaccctgactcctctgatccacaaacatgttgcaccgtctcatcactgaagggctgagccgctcctcagtctgtgagtctgcagtggtcacagcacgcatgagaggcagactctgaacctgcacaaagccagagccttgggtgatgtggggacctcgcaagagttactgggaatggagatcctggccttgggacagagggagtggggctgcacaggagtcccccatcatcctggtggtgggggagcctatgcaggaagtcaagaagtctcttcagcacaaaccagttaaggcgaggggctcttacctggcctgactgctgggggtggggtgggggtcacccctgct

SEQ ID NO: 16186 - RNA, 2941 nt, Homo sapiens
  source 1..2941: mol_type = other RNA
gctgggattacaggcatgagcctctgtgcctggccaaaagtaggtcttcctgaagtcagcacagtttagaagtcagtcttcaatcttccaaataccacaatttttctttaaataaacatgcattcagaggagaactcaaatggaagaaaaacatgcataatcctaccagtaaattttccaaaactcctaatgcagttttttatgacttgaacttatcaatatagtattttgagatgcactgaaatatttagagaaatttggttgtaaccaatgacaactaaatacacttgcctgttttttcaaaaaaataaaggagtaataatttggtgaagttttcagagtggttgccagtcactgctaggaaagatgtcgttagcttctggcaagtcagaaaagtaggatgaagaatctgatcttgaaatatcttcttttttttttctttttcatcttgctgcttttcttcccgacactaaaagatttgtcttcctgacaaattgatgtagaaagcagcacacctgtgacccaaagagaaacttgaaaatgtgtgtccttaccatgcgttcagatattgtagctttagtgtaagttttagaaacgatttcagtaaaacatgcctcttctaggtcatcctgggatcagctcagggtgaggccctggggaacacaggatgtggtctgtgaacaaaaggaatatttgtgcccgcaattgactgcagtggggaagggctctgatttcaaacagaatatttcaaaaggcattgcttactcttggtcttagagctatgctctgactggctgtattccaaagaagtccagaaagagaaggcgatatttcaaagtattatttctttgttgcattcttcactccctgtaatcacatgtttctgtgtattatcatgtgtttaatgtctgtctggccagctgctctccataagggcagggctcttctcttgcccacagtgcctcactctgcccttccctgcttcagtgaggcctggggagccatcaggggcctgtggacatcgttctggatgagttttgttcattttgcacgaggtcttgaatttctttccaaggttggcaggtggaggccaatggggtgattctgacccgatatgatattgtgcgcgatcagcctgccagtcaaccacaggctcccacagccctgaggttggagcttcagagagaagcaattttgacaaaccagggctgaaggagtggaatgtattttggttggaatccatgactttttattaccaccgattaaacaggaaacaaacattttgagcaggttccaatcctcagctgaatgtggctgcgccatccatgtatggggacactcggtctccagccattctaccgggacacgggagggccctgggaggcacccacctgcctcagtgttccagttactaaaaatgagactggattttaaggcagtggatctggcctggctttctgtgtccagggtgggctggaactggatctgattaggtgggtctaggcactgacagcacctgatttggtgtgcacctgctgaggacgtgtgcaggtggggaaggaggggcccacatggaagaggggtgcatgatgcatgagctgaaaggcggcatgtggaggctgaagcccagtgggctgaggattctgcagtggggtggcctgatgaagtgggcactctgaagtgtgtccacctgccgtgacctgctaaagcacagtggacccactgcctcggtggacaccttgaagcattgctgttctgaaggcaccttggcctaaccagatgatgacagggcccaccccaggggcccctgaggccctgtggtcacccctaacaaggacgcttgggctgattattttcatgaagtgtcgggatgggcactgcttctcctgctggacttgaggtggttgggaagggtttcccctaatgttctgcctgaaatgccccagccagatgtaacacctgcctccctaactctctcttcctactcccatcccttgctccttccacttgtgtaactacagtatagggtggcataagcaaagtcttcctagaggatggacacctttgagatggcaactatatcttctttataagcctacacccttctgtgtagagcttattccacacatccatccacccacctccccacctacccatccatccatccatctgcacattcatacattcatctgtctgtcatcaatccatccatccatccaacaaatgtaaattatgcacctaccatatgccaagcactgggcttggtactgagagtgaaagaacataaatggaccctgctagaaccccagtgcctggtacacagtagatgctcagatatgttcactgaataaatgcatgacaaaatccccatcttcatgctatagctcacaaagaattggaaaaaggagggctttggaattttgggagcagtcacttgtccagctcacatggactgcctctggaggccccttttttggtggaaccaacaggagaaaagaggctgcacctctgagaccatgaccaagttccgtgaaacaatgaagccagcagtaaggcatttcccttgccacccgtccagctgccagagcgtggctgagactcgagagtttagaataatgaatttcatccccactgtgctggtgacagacagagccggagatctcaggaaagtacatgtgaggctgagagtggaggtgggcagatttccaggggtgagtgagacaaaggagaggtctgtgtgaggggccgcccctgagggaagtgaataacatccttggcagtgattagctaaccacatcaagctgggaggaagagggagtggggaggccttctgcctgcgggcagagtagctcccatcttccacctgtggcaagcccaattacattgtcttcagagccaggaaaaagctggaatgtttccctaatgaaaatgcttttgctat

SEQ ID NO: 16187 - RNA, 1010 nt, Homo sapiens
  source 1..1010: mol_type = other RNA
gctgggattacaggcatgagcctgtaatcccagcactttgggaggccatggcaggcagatcacctgaggtcaggagttcgagaccaggctggccaacatggcgaaaccctgtctctactaaaaatacaaaaagtagcctggcgtggtggcgtgcactggtaatcccagctactcaggaggctgaggcacaagaatcacttgaacacaggaggtggaggttgcagtgagtctagataatgccactgcactccaggctgggcaacagagtgagactctgtctcaaaaaaacaaaaacaaaaaataaataaataaataaataaaaacatgaagattcttaagccaaagaaaaagaaaaagaaatttgaggagaaaataaatttttaaaaaaattatttcaaattagattttacaaactaaaacattattggtgaatttggttaaagggtatctaagagttcctttcattattcttgcatctgcatcttttctgtaggttgaaattattcccccccgccctccagaaaaaaagtaggtaatggaagtcctgggaagatgaagagaggcttctctggccttgagaaagagccagtatatttattcatacattcaacatatatgtattaaatgcctaccttgtgccaagcattatcctcgtttctggggatgtggacttgaatgggtggggtgcagtggtgcagacctgtagtcccagctgcttggtaggctgaggtgggagaattgctcgagcccagaagttcaagtccagcctgggcaacataatgcgacccgtcctcaaggtgttcgcagccgccgccgcaccgccatgccgccatcactctccaacgccagcgctgcctctggctcgcagagctccagctgaaggataagggaggtaaataaggaagcctctataccatggcttgtacaaagcggactgcctgcaaatcgaccgtaaagcagccaggaagcaactgggtacaaaagccgctcacaagagtgcgccctctact

SEQ ID NO: 16188 - RNA, 5768 nt, Homo sapiens
  source 1..5768: mol_type = other RNA
gctgggattacaggcatgagcctgtaatttctggccatgcctggccagaaatcagaagttgcaagagtaaatattcagtgttgtactacagtcagtttccattttgtgatttttgtcttataccaccatttatacctctgcactccctcttcttattctgcccatctggccaagctgataatgtccgtgttccctcctttggcactagatggaagttcaaatcacgtgtgggatcctcaccccaacccacccttttattaaaggttattaccataacaccccaagcaagttatttatccctgctctctcaagccattttggaccagtttgggaagtcaatcctgcttctcacagaaagcctcattatgcaatacacatttccctaaaacttcattgttcagcatcctcattttccatatctaaaccaaactgtaaatggagttcaatacacttcctgtggagaggtgacaaattaacattaccaaaaacatgataaggctaaatttatgaaacttctagtttacctacaaaaacaaaatttccattatatatgttcatttttaagaggaaactcatgaatattagtcttgtcaaattatgtgagcatagcattcttagtgttatttttgttattctgcactatttataatttcataatttttttttttgagacggagtctcactttctcgcccaggctggagtgcagtggcaatctcggctcactgcaacctccacctcctgggttcaagtgattctcctgcctcagcctcccgagtagctgggattacaggcgcatgccaccacatccaaccaatatatatatatttggtattttttagtagagatggggtttcactgtgttggccagggtggtctcgattttctgaccccatgatccacccgccttggcctccctaagtgctgggattacaggtgtgagccaccacacccagccaatatttttcatacaattgttttttttgagacagggtctcgctctgtcacccaggctggagtgcaatggcgcgatcttggctcactgcaacctctgcctccaggctcaagtgatccacctgcctcagtctccctgaggagctgggactacaggcatgagccaccctgcctgggtaatatttctattttttttgtagagacagggttttgccatgttgtcctggctggttcaaactcctggactcaagtgacccccctgccttgggctctcaaagtgctaggattacaggcatgaaccaccacacccagcccatacactttctatatttgtattttcacttcatgtaaataaagatgcatgccatagttatttagcacacaagcatgtaaaaatataatatggtatatattcaccaacactgtggcagctttcagagtgtaagagtatgaaaactgcactttctatgggattttcattatatccatataaatattctaaggcagagtgtagagagaataattcaagtgcagagtatgattacattttcccaaaattgtatgttgattccacaaagaaaaaaaaaattgttctacatcctccaacctaaaagactgagtgtattgttattatctgctatgaagtatcctactgaggtaggataaaatgatgttggtacaaagaatgtgatttgtttatagttataagaaaacgttgaattttttttagcaaaacattatgtctgtgacacattcttaataaaactgtagcaaaatgtaattccagcaattagtgtgaattctactaaaaacaaaacaaaacaaaaaaaaccatggtattctggtttttctgaccaagctctccactctaataactgttacctcttcaatttcaaaaataagcctatttttcatcaatctctgctataaaacagctattgccattcagtagagaaagtggcaaccatttcccctgcactattcccatcacataatcagtcactaataacttattactctcctctcataaaaattccagtgtcctgaggtcttggcctgctcaatgcaggtagagccttacttccctaaaacccatggtgtctttctctcagaaaagcaccctgaacacaatcagtatgatgattgatatcatagttttacattattttctgccccaaaaccatggtctctcaattgagagaatatttaattttacaaggcagagtcctccttcttcaataaacatggataaaaatgatcctcatgtaatgaagtaagcctttccatactgtggttctttcccagataggcaccacgaaaggtgcttaaggatgcaaaatagccacagatccatagttcaggttgaaagtcacaaacagtagcctttttgagaaacctcaaacaatggaataaaagattttataacctgaaggtaagtagccatttccaaatgtcctttgacctttgaaatatataatgtcttaagttttaccatattggaacgtgtaattattgtgcagtttatcattttaaaagtgaatcaaagaactagagactgagtcactctttgtatgaatcctcacctacagttacagtcttagagtaagagcttcaggatgctcttacacattacatttgtgtggttccatcaaatacgtagattttaatgcctgcaaagctgtgaggcctgaataaagcctctgtcacacacagtacatttatgtgatttctcattattatggactcttggatgtctattaatacttgaactcatgaggagtttgccacagtcattgcattttttttttttcctttaagatggagttttgctctttttgcccaggatggagtgcattggcacgatcttggctcactgcaacctccgcctcctgggttcaagtgattctcctgcctcagcctcctatatagctgggattacaggcgcacgccaccaggcctagctaattgtgtacttttagtagaaatggggtttcgccatgttggtcaggctggtcttgaactcctgacctcaggtgatccacctgcctcggactcccaaagtgttgggattacaggcatgagccactgcacccagccagtcattgcattttcaaggaatctctcaggcataaattctctgacgttgtcaaaggaatgaattctaactgcaaaagttaccaccttcatttgtaaggtttctctccactatgaattctgtgatggcttgcaaggtttgaactctgactttagaactttccacacgttacatttgtaaggtttcccaccagtatggattgtctgatgggtagttaggcttgaacagatactaaagggtttcccacactcatatggtttctctccggtatgaattctctgatgccttgcaagttttgaagtttgactaaaggctttgccacactcattacacttgtaaggtttctctccagtatgaattccccgatgtcttgcaaggtgtgaattctgagtgaagaccttcccacactcattgcatttgtaaggtttttttccagtatggattgcctgatgggtagttaggcttgaacggacactaaaggctttcccacactgattacactcatatggtttctctccagtatgaactctctgatgccttgcaagctttgatgtttgactaaaggctttgccacattcattacactggtaaggtttacctccagtatgaactctccgatgtcttgcaaggtgtgaattctgagtgaagaccttgccacactcattacatttgtaaggtttttcaccagtatggatgacctgatgggtagttaggtttgaatgttcactaaaggctttgccatactcattatacttgtaaggtttctctccagtatgaattcgctgatgccttgaaaggtatgaattatgcctaaagaccttgccacattcattacatttataaggtttctctccagtatgaattccccgatgtcttgcaaggtgtgaattctgagtgaagaccttgccacactcattacatttgtaaggtttttctccagtatggatgacctgatgggtagttaggcttgaatacacactgaaggctttgccgcactcattacacatataaggcttcactccagtatgaattctttgatgatttgcaaggtgtgaattttgagtgaagaccttgccacattcattacatttgtaaggcttttctccagtatggatgacctgatgggtagttaggtttgaatgtgctctaaaggctttgccacactcattacacttataaggtttctctccagtatgaattagctgatgccttgcaaggtgtgaattacgcctaaagaccttgccgcattcatgacatttgtaaggcttttctccggtgtgaattaccagatgaatagctaggcttgaacgaacaccaaaggctttgccgcactcattacacttgtaaggtttctctccagtgtgaattctccagtgatttgtaaggtgtgaattttgagtgaagaccttgccacattcattacatttgtaaggtttttctccactgtgggttgcctgatggatagctaagcttgaacgagctctaaaggctttcccacactcattacacttgtaaggtttctctccagtatgaattcctcgatgtcttacaaggtgtgaattctgagtgaagaccttgccacattcgttacatttataaggtttctctccagtgtgaattttctgatgttgtgagagttgtgaatttcgactaaagaccttaccacactcattacatttgtaacgtttttcgccagtatggatcacctgatgggtagttaggtttgaacgtgttctaaaggctttgccacactcataacatttgtaaggtttctctttagtatgacttctctgatgacttgcaaggtgtgaattttgaggaaagaccatgccacatccattagatttgtaagggcttccccaattatttgctttttgcccctgtgtgagtaataaagaagagataaaatctttgagatatttcttagaaatgtgggttttgacattataaggcatttgttgaggtggtgaaactgaggaattattgttgaaagacttctcaacctgattacattcataaattttcccttcatattgaaaaagctgcagttcaggcagatgtgactgaaggcttaatccaagctgatttttaataagcttgtttcttgcatctcttttatcatgttcatctcttccatgagtgagattgccttcttgggtcaaaagcactcctttgtaatttccttcagcatctctgcattgatactcaaggccatgtgtatttttctggacttccctgaaggaacatccttcaatgtcttggctttcctgtctttccaacatcactgtttggaatacttctcctgtattactcttccctttgtgtagtaaatctttcattacaaattcggaagagagagctgtgatcacagctttgatccattcccatccatctgggtttcctgctatttgtacttggctctccaaagtgaaaggctccttcccttgctccaacatagagataatactgaggtcaaaacaagagattcccagggaggccaggttcctataattctccaacatcacgtccctgtacaaagtcctctgagcggggtccaggcatgtccactcctcctgagagaattctatagccacatccctgaatgtcacctgtccctgggtgagagccatgcctgacttgtctttctttcctcttcctcttcttcaagggttcttcgctcggcggcgtcacccgcacccaacacgatccgcttccggaact

SEQ ID NO: 16189 - RNA, 6100 nt, Homo sapiens
  source 1..6100: mol_type = other RNA
gctgggattacaggcatgagcctgtaatttctggccatgcctggccagaaatcagaagttgcaagagtaaatattcagtgttgtactacagtcagtttccattttgtgatttttgtcttataccaccatttatacctctgcactccctcttcttattctgcccatctggccaagctgataatgtccgtgttccctcctttggcactagatggaagttcaaatcacgtgtgggatcctcaccccaacccacccttttattaaaggttattaccataacaccccaagcaagttatttatccctgctctctcaagccattttggaccagtttgggaagtcaatcctgcttctcacagaaagcctcattatgcaatacacatttccctaaaacttcattgttcagcatcctcattttccatatctaaaccaaactgtaaatggagttcaatacacttcctgtggagaggtgacaaattaacattaccaaaaacatgataaggctaaatttatgaaacttctagtttacctacaaaaacaaaatttccattatatatgttcatttttaagaggaaactcatgaatattagtcttgtcaaattatgtgagcatagcattcttagtgttatttttgttattctgcactatttataatttcataatttttttttttgagacggagtctcactttctcgcccaggctggagtgcagtggcaatctcggctcactgcaacctccacctcctgggttcaagtgattctcctgcctcagcctcccgagtagctgggattacaggcgcatgccaccacatccaaccaatatatatatatttggtattttttagtagagatggggtttcactgtgttggccagggtggtctcgattttctgaccccatgatccacccgccttggcctccctaagtgctgggattacaggtgtgagccaccacacccagccaatatttttcatacaattgttttttttgagacagggtctcgctctgtcacccaggctggagtgcaatggcgcgatcttggctcactgcaacctctgcctccaggctcaagtgatccacctgcctcagtctccctgaggagctgggactacaggcatgagccaccctgcctgggtaatatttctattttttttgtagagacagggttttgccatgttgtcctggctggttcaaactcctggactcaagtgacccccctgccttgggctctcaaagtgctaggattacaggcatgaaccaccacacccagcccatacactttctatatttgtattttcacttcatgtaaataaagatgcatgccatagttatttagcacacaagcatgtaaaaatataatatggtatatattcaccaacactgtggcagctttcagagtgtaagagtatgaaaactgcactttctatgggattttcattatatccatataaatattctaaggcagagtgtagagagaataattcaagtgcagagtatgattacattttcccaaaattgtatgttgattccacaaagaaaaaaaaaattgttctacatcctccaacctaaaagactgagtgtattgttattatctgctatgaagtatcctactgaggtaggataaaatgatgttggtacaaagaatgtgatttgtttatagttataagaaaacgttgaattttttttagcaaaacattatgtctgtgacacattcttaataaaactgtagcaaaatgtaattccagcaattagtgtgaattctactaaaaacaaaacaaaacaaaaaaaaccatggtattctggtttttctgaccaagctctccactctaataactgttacctcttcaatttcaaaaataagcctatttttcatcaatctctgctataaaacagctattgccattcagtagagaaagtggcaaccatttcccctgcactattcccatcacataatcagtcactaataacttattactctcctctcataaaaattccagtgtcctgaggtcttggcctgctcaatgcaggtagagccttacttccctaaaacccatggtgtctttctctcagaaaagcaccctgaacacaatcagtatgatgattgatatcatagttttacattattttctgccccaaaaccatggtctctcaattgagagaatatttaattttacaaggcagagtcctccttcttcaataaacatggataaaaatgatcctcatgtaatgaagtaagcctttccatactgtggttctttcccagataggcaccacgaaaggtgcttaaggatgcaaaatagccacagatccatagttcaggttgaaagtcacaaacagtagcctttttgagaaacctcaaacaatggaataaaagattttataacctgaaggtaagtagccatttccaaatgtcctttgacctttgaaatatataatgtcttaagttttaccatattggaacgtgtaattattgtgcagtttatcattttaaaagtgaatcaaagaactagagactgagtcactctttgtatgaatcctcacctacagttacagtcttagagtaagagcttcaggatgctcttacacattacatttgtgtggttccatcaaatacgtagattttaatgcctgcaaagctgtgaggcctgaataaagcctctgtcacacacagtacatttatgtgatttctcattattatggactcttggatgtctattaatacttgaactcatgaggagtttgccacagtcattgcattttttttttttcctttaagatggagttttgctctttttgcccaggatggagtgcattggcacgatcttggctcactgcaacctccgcctcctgggttcaagtgattctcctgcctcagcctcctatatagctgggattacaggcgcacgccaccaggcctagctaattgtgtacttttagtagaaatggggtttcgccatgttggtcaggctggtcttgaactcctgacctcaggtgatccacctgcctcggactcccaaagtgttgggattacaggcatgagccactgcacccagccagtcattgcattttcaaggaatctctcaggcataaattctctgacgttgtcaaaggaatgaattctaactgcaaaagttaccaccttcatttgtaaggtttctctccactatgaattctgtgatggcttgcaaggtttgaactctgactttagaactttccacacgttacatttgtaaggtttcccaccagtatggattgtctgatgggtagttaggcttgaacagatactaaagggtttcccacactcatatggtttctctccggtatgaattctctgatgccttgcaagttttgaagtttgactaaaggctttgccacactcattacacttgtaaggtttctctccagtatgaattccccgatgtcttgcaaggtgtgaattctgagtgaagaccttcccacactcattgcatttgtaaggtttttttccagtatggattgcctgatgggtagttaggcttgaacggacactaaaggctttcccacactgattacactcatatggtttctctccagtatgaactctctgatgccttgcaagctttgatgtttgactaaaggctttgccacattcattacactggtaaggtttacctccagtatgaactctccgatgtcttgcaaggtgtgaattctgagtgaagaccttgccacactcattacatttgtaaggtttttcaccagtatggatgacctgatgggtagttaggtttgaatgttcactaaaggctttgccatactcattatacttgtaaggtttctctccagtatgaattcgctgatgccttgaaaggtatgaattatgcctaaagaccttgccacattcattacatttataaggtttctctccagtatgaattccccgatgtcttgcaaggtgtgaattctgagtgaagaccttgccacactcattacatttgtaaggtttttctccagtatggatgacctgatgggtagttaggcttgaatacacactgaaggctttgccgcactcattacacatataaggcttcactccagtatgaattctttgatgatttgcaaggtgtgaattttgagtgaagaccttgccacattcattacatttgtaaggcttttctccagtatggatgacctgatgggtagttaggtttgaatgtgctctaaaggctttgccacactcattacacttataaggtttctctccagtatgaattagctgatgccttgcaaggtgtgaattacgcctaaagaccttgccgcattcatgacatttgtaaggcttttctccggtgtgaattaccagatgaatagctaggcttgaacgaacaccaaaggctttgccgcactcattacacttgtaaggtttctctccagtgtgaattctccagtgatttgtaaggtgtgaattttgagtgaagaccttgccacattcattacatttgtaaggtttttctccactgtgggttgcctgatggatagctaagcttgaacgagctctaaaggctttcccacactcattacacttgtaaggtttctctccagtatgaattcctcgatgtcttacaaggtgtgaattctgagtgaagaccttgccacattcgttacatttataaggtttctctccagtgtgaattttctgatgttgtgagagttgtgaatttcgactaaagaccttaccacactcattacatttgtaacgtttttcgccagtatggatcacctgatgggtagttaggtttgaacgtgttctaaaggctttgccacactcataacatttgtaaggtttctctttagtatgacttctctgatgacttgcaaggtgtgaattttgaggaaagaccatgccacatccattagatttgtaagggcttccccaattatttgctttttgcccctgtgtgagtaataaagaagagataaaatctttgagatatttcttagaaatgtgggttttgacattataaggcatttgttgaggtggtgaaactgaggaattattgttgaaagacttctcaacctgattacattcataaattttcccttcatattgaaaaagctgcagttcaggcagatgtgactgaaggcttaatccaagctgatttttaataagcttgtttcttgcatctcttttatcatgttcatctcttccatgagtgagattgccttcttgggtcaaaagcactcctttgtaatttccttcagcatctctgcattgatactcaaggccatgtgtatttttctggacttccctgaaggaacatccttcaatgtcttggctttcctgtctttccaacatcactgtttggaatacttctcctgtattactcttccctttgtgtagtaaatctttcattacaaattcggaagagagagctgtgatcacagctttgatccattcccatccatctgggtttcctgctatttgtacttggctctccaaagtgaaaggctccttcccttgctccaacatagagataatactgaggtcaaaacaagagattcctgccagggaggccaggttcctataattctccaacatcacgtccctgtacaaagtcctctgagcggggtccaggcatgtccactcctcctgagagaattctatagccacatccctgaatgtcacctgtccctgggtgagagccatgcctgacttgtctttctttcctcttcctcttcttcaagggttcttcctgaggtcaggagttcgagatcagcctgggcaacacggtgaaaccccgtctctactaaaaatacaaaattagccgggcgtggtggcacatgcctgtaatcccagctactcgggaggctgaggcaggagaatcgcttgaacctgggaggcggaggatgcggtgagccgaaatcgcgccattgcactccagcctggacaacaagagtaaatctccgtctcaccaaaaaaaaaaaaaaagaaaaaaaaaaaggtctgtagcgagcccgggaactggctgcggaaacggggcacggcggttcgcaagtttaatccatactgagggacactcacgctcggcggcgtcacccgcacccaacacgatccgcttccggaact

SEQ ID NO: 16190 - RNA, 5771 nt, Homo sapiens
  source 1..5771: mol_type = other RNA
gctgggattacaggcatgagcctgtaatttctggccatgcctggccagaaatcagaagttgcaagagtaaatattcagtgttgtactacagtcagtttccattttgtgatttttgtcttataccaccatttatacctctgcactccctcttcttattctgcccatctggccaagctgataatgtccgtgttccctcctttggcactagatggaagttcaaatcacgtgtgggatcctcaccccaacccacccttttattaaaggttattaccataacaccccaagcaagttatttatccctgctctctcaagccattttggaccagtttgggaagtcaatcctgcttctcacagaaagcctcattatgcaatacacatttccctaaaacttcattgttcagcatcctcattttccatatctaaaccaaactgtaaatggagttcaatacacttcctgtggagaggtgacaaattaacattaccaaaaacatgataaggctaaatttatgaaacttctagtttacctacaaaaacaaaatttccattatatatgttcatttttaagaggaaactcatgaatattagtcttgtcaaattatgtgagcatagcattcttagtgttatttttgttattctgcactatttataatttcataatttttttttttgagacggagtctcactttctcgcccaggctggagtgcagtggcaatctcggctcactgcaacctccacctcctgggttcaagtgattctcctgcctcagcctcccgagtagctgggattacaggcgcatgccaccacatccaaccaatatatatatatttggtattttttagtagagatggggtttcactgtgttggccagggtggtctcgattttctgaccccatgatccacccgccttggcctccctaagtgctgggattacaggtgtgagccaccacacccagccaatatttttcatacaattgttttttttgagacagggtctcgctctgtcacccaggctggagtgcaatggcgcgatcttggctcactgcaacctctgcctccaggctcaagtgatccacctgcctcagtctccctgaggagctgggactacaggcatgagccaccctgcctgggtaatatttctattttttttgtagagacagggttttgccatgttgtcctggctggttcaaactcctggactcaagtgacccccctgccttgggctctcaaagtgctaggattacaggcatgaaccaccacacccagcccatacactttctatatttgtattttcacttcatgtaaataaagatgcatgccatagttatttagcacacaagcatgtaaaaatataatatggtatatattcaccaacactgtggcagctttcagagtgtaagagtatgaaaactgcactttctatgggattttcattatatccatataaatattctaaggcagagtgtagagagaataattcaagtgcagagtatgattacattttcccaaaattgtatgttgattccacaaagaaaaaaaaaattgttctacatcctccaacctaaaagactgagtgtattgttattatctgctatgaagtatcctactgaggtaggataaaatgatgttggtacaaagaatgtgatttgtttatagttataagaaaacgttgaattttttttagcaaaacattatgtctgtgacacattcttaataaaactgtagcaaaatgtaattccagcaattagtgtgaattctactaaaaacaaaacaaaacaaaaaaaaccatggtattctggtttttctgaccaagctctccactctaataactgttacctcttcaatttcaaaaataagcctatttttcatcaatctctgctataaaacagctattgccattcagtagagaaagtggcaaccatttcccctgcactattcccatcacataatcagtcactaataacttattactctcctctcataaaaattccagtgtcctgaggtcttggcctgctcaatgcaggtagagccttacttccctaaaacccatggtgtctttctctcagaaaagcaccctgaacacaatcagtatgatgattgatatcatagttttacattattttctgccccaaaaccatggtctctcaattgagagaatatttaattttacaaggcagagtcctccttcttcaataaacatggataaaaatgatcctcatgtaatgaagtaagcctttccatactgtggttctttcccagataggcaccacgaaaggtgcttaaggatgcaaaatagccacagatccatagttcaggttgaaagtcacaaacagtagcctttttgagaaacctcaaacaatggaataaaagattttataacctgaaggtaagtagccatttccaaatgtcctttgacctttgaaatatataatgtcttaagttttaccatattggaacgtgtaattattgtgcagtttatcattttaaaagtgaatcaaagaactagagactgagtcactctttgtatgaatcctcacctacagttacagtcttagagtaagagcttcaggatgctcttacacattacatttgtgtggttccatcaaatacgtagattttaatgcctgcaaagctgtgaggcctgaataaagcctctgtcacacacagtacatttatgtgatttctcattattatggactcttggatgtctattaatacttgaactcatgaggagtttgccacagtcattgcattttttttttttcctttaagatggagttttgctctttttgcccaggatggagtgcattggcacgatcttggctcactgcaacctccgcctcctgggttcaagtgattctcctgcctcagcctcctatatagctgggattacaggcgcacgccaccaggcctagctaattgtgtacttttagtagaaatggggtttcgccatgttggtcaggctggtcttgaactcctgacctcaggtgatccacctgcctcggactcccaaagtgttgggattacaggcatgagccactgcacccagccagtcattgcattttcaaggaatctctcaggcataaattctctgacgttgtcaaaggaatgaattctaactgcaaaagttaccaccttcatttgtaaggtttctctccactatgaattctgtgatggcttgcaaggtttgaactctgactttagaactttccacacgttacatttgtaaggtttcccaccagtatggattgtctgatgggtagttaggcttgaacagatactaaagggtttcccacactcatatggtttctctccggtatgaattctctgatgccttgcaagttttgaagtttgactaaaggctttgccacactcattacacttgtaaggtttctctccagtatgaattccccgatgtcttgcaaggtgtgaattctgagtgaagaccttcccacactcattgcatttgtaaggtttttttccagtatggattgcctgatgggtagttaggcttgaacggacactaaaggctttcccacactgattacactcatatggtttctctccagtatgaactctctgatgccttgcaagctttgatgtttgactaaaggctttgccacattcattacactggtaaggtttacctccagtatgaactctccgatgtcttgcaaggtgtgaattctgagtgaagaccttgccacactcattacatttgtaaggtttttcaccagtatggatgacctgatgggtagttaggtttgaatgttcactaaaggctttgccatactcattatacttgtaaggtttctctccagtatgaattcgctgatgccttgaaaggtatgaattatgcctaaagaccttgccacattcattacatttataaggtttctctccagtatgaattccccgatgtcttgcaaggtgtgaattctgagtgaagaccttgccacactcattacatttgtaaggtttttctccagtatggatgacctgatgggtagttaggcttgaatacacactgaaggctttgccgcactcattacacatataaggcttcactccagtatgaattctttgatgatttgcaaggtgtgaattttgagtgaagaccttgccacattcattacatttgtaaggcttttctccagtatggatgacctgatgggtagttaggtttgaatgtgctctaaaggctttgccacactcattacacttataaggtttctctccagtatgaattagctgatgccttgcaaggtgtgaattacgcctaaagaccttgccgcattcatgacatttgtaaggcttttctccggtgtgaattaccagatgaatagctaggcttgaacgaacaccaaaggctttgccgcactcattacacttgtaaggtttctctccagtgtgaattctccagtgatttgtaaggtgtgaattttgagtgaagaccttgccacattcattacatttgtaaggtttttctccactgtgggttgcctgatggatagctaagcttgaacgagctctaaaggctttcccacactcattacacttgtaaggtttctctccagtatgaattcctcgatgtcttacaaggtgtgaattctgagtgaagaccttgccacattcgttacatttataaggtttctctccagtgtgaattttctgatgttgtgagagttgtgaatttcgactaaagaccttaccacactcattacatttgtaacgtttttcgccagtatggatcacctgatgggtagttaggtttgaacgtgttctaaaggctttgccacactcataacatttgtaaggtttctctttagtatgacttctctgatgacttgcaaggtgtgaattttgaggaaagaccatgccacatccattagatttgtaagggcttccccaattatttgctttttgcccctgtgtgagtaataaagaagagataaaatctttgagatatttcttagaaatgtgggttttgacattataaggcatttgttgaggtggtgaaactgaggaattattgttgaaagacttctcaacctgattacattcataaattttcccttcatattgaaaaagctgcagttcaggcagatgtgactgaaggcttaatccaagctgatttttaataagcttgtttcttgcatctcttttatcatgttcatctcttccatgagtgagattgccttcttgggtcaaaagcactcctttgtaatttccttcagcatctctgcattgatactcaaggccatgtgtatttttctggacttccctgaaggaacatccttcaatgtcttggctttcctgtctttccaacatcactgtttggaatacttctcctgtattactcttccctttgtgtagtaaatctttcattacaaattcggaagagagagctgtgatcacagctttgatccattcccatccatctgggtttcctgctatttgtacttggctctccaaagtgaaaggctccttcccttgctccaacatagagataatactgaggtcaaaacaagagattcctgccagggaggccaggttcctataattctccaacatcacgtccctgtacaaagtcctctgagcggggtccaggcatgtccactcctcctgagagaattctatagccacatccctgaatgtcacctgtccctgggtgagagccatgcctgacttgtctttctttcctcttcctcttcttcaagggttcttcgctcggcggcgtcacccgcacccaacacgatccgcttccggaact

SEQ ID NO: 16191 - RNA, 7341 nt, Homo sapiens
  source 1..7341: mol_type = other RNA
gctgggattacaggcatgagcctgtgttctcccctctcttccaataatgtgtattcaacaaggccttcaggtgatgctgatgctgtctgaaagccactgctctccagcatgtggtctctgaaactttacttaggagtatgcatattaaaatatatatataacttaacactatgctactacaaagggcaaaataattcactttattgtactttattttagaataattaagacaaggataggcttcaatgaaattttgctttgatgttacatggtctgactgacactggatttcttcataagaaaaataaatgtgaaagctattccaagtaagcaaatggtggcaaaaacaatctaaagaattggttttagccaggcatggtggctcatgcctgtaatcccagcactttgggaggccagggcgggcagattacttgagctcaggagttcaagagcagcctggccaacatggtgaaaccccatctctactaaaaacacaaaaattaggcaatatagcaagaccccatctctaccaaaaatacaaaaaaactaatcaggaatgggggcacatgccagtagtcccaactactcaggagactgaggtgggaggatggcttgagcttgggaggttgcagtgagccaagatcctgccactgcactccagcctgggtgacagagtgagaccccatctcaaaaaaaaaaaaagaatttcatctcatgtcaaaaataagactcttggacagaaatcttctgcctgccttccaaggacccactgaaattaatggatactctcacatgactgactttattattaaatacttgctgtaatcacaactaggcataggaaaatcaagtagagaaatactgaatgcctagcatacaacgatctaagtgaaagttaataaaagtagctcttcagaaagacatctcatgtaaaattaaatttaaaactaaaaatttcatgaagtgacctgttaagagtttcaatttagaagctttacttttctaattttaaaatatcatgaatgaaatggtgtcttcatctaggtgcttctccatcaaaatccctagctcaaaaataaaaatcatgtttgtgtcaccccagattcaaaatgctgttattggaaatgttaccatttcacatgaacattccagtaaatatgcacatagagggtactcattacttttggttggtaatttttccttaaatatatttcaatgatttcattgtttgacattttcatagttaacgtatactgaatacagaaaattttgtaggaaaacactattttttaaatgtagtaacattaaaatattaaaatatcccgtttattaaaggctcttaagatttaaagaaaaatttcctgtgcacatacaatgtacctatgaaatactgtattattagttattgtacaggcaaatgaggctgttactataaaaaaaatgtggtgtctaaaaattgcaagtctatgtgaaaaatcaacctcaatttatctaaatgggatttgggggacacggcagactattaaaatagaactcaaacttcaaattctgtaaactgaacatctcattaatgccacttcaccatttaaaaaagtcagcacacaatgttagctatgtaagtttatctgcagatgttacaggtaattatttctgttaactcctcctaaaatattatttagtaataaagaatatttcaaaaggagagtaggtagaaacgaagatcataactatacttacttaatatgaaaatgacatttcatttatttgctaatatgtggaaaaaaattttctaattaattcctcctttatccttctttaaaaacattttatttcttcaaccagcacactgaggattagtgctatgggtattaccacagtgccctgtgaaaagacttggcttccagagaagtcataccttgcataccctggagtcatacctcaaattggctctgcatgattgattttacagcgggcattaaaattcttctgaaacaaggctgtgtacctttgagaacattcacatttaaccttgtgagctcacttctacaagaacaatgaacttatttgtcagctgccagggggaaaatcagcttaatgtaaagaattaattaaatcaggttgacagaagccaatatctcaatgtttttaaattaaaatttatttaaaggaataagtatgggtgcattacataaacctaatggttcttctaagcttcaaaaagcattcatttcaaaagtattcactttttttttttttgagacggagtctcgctgtcgcccaggctggagtgcaggggcacgatctcggctcactgcaggctccgcctcccgggttcacgccattctgctgcctcagcctcccgagcagctgggactacaggcgccgccaccacgcccggctaattctttgtatttttagtagagacggggtttcactgtgttaaccaggatggtctcgatctcctgacctcgtgatccgcccgcctcggcctcccaaagtgctgggactacaggcgtgagccaccacgcccggcccaaaagcatttactgttaaggctgcctcatttttcagctttgttgtagttgagattctgatgttcacctaacaaagtccctgacaaaacagacttccttcaatccaggtcataatttgaaacgttatacaataatgagatttaagtgatgaatggaaagaaaagaaggagactgaaaagatatcagaaatttctatttgtttttagattcagaaaaatataattacaggccaacatgggtctgacagagaggaaggacgtcagcagttacttgaatgtaaccccttcccagcatttccaaagacctgcaatgtgctcattgtgatccaagggccttgttacctagtttctaggtgatctacagaattgaaacaacccagcacaactttatttcttgagaagatgaacccttaactatgaaggtgcagaaaggaagtcttcaactgctcactcaccatggctacagtattcaaatgcaacaatcattcagataaataaaacctgtgagaaaaagcaaacaggtgggcaagcaaagcggcagtgattcatactttcagttaaccaattgaacagtggtgcttccttctgaagaagttgttcattgatttttgttttttaagaaacagaaaagcagcagtataatgaaagaagattggctgaagatctatccagcctgttaactacggcttagtacttccagaatcctgagtaacaacacatgacctgtgtgatgataagagcacagaacacatgaacaaccaaaagattctaagctcagcctctttccctatagtatttacagaataattttaaatttcagtttcacctccactacttcaacgattttaccctgtaaattgctgaaggtctttgtgaactgtcgaacagcaaaaacaaaaagtagaggtatctagattataaacttcaaccaaaagtagtccttgagtaattaaaatgttacttcattatgttctttttaaaagaaaattcctcagaagtccacattctttacatgccttcaccctgttgagctaaacaggtcaaaagtataataaactcaacattatttttaacttgcgttattggtggtgccaaatgagaaaagagctgtttttgccactttgggctggatgattaaaaaaaaaaaaaaaaaaaaagagagctgtttgtattttaaatttaatatcataaacaatttttaaaggtaatataatatagaagttctcagaatgaaacaaaaggaaggctaaacttcattttagactcatggtaacaccaaagcaattttaagaatgtgaataggaagctaaacactgcaaagagaattcttaaaaatcagattagttaagaaattttgaagagaactaaactcttcacagcaaacttgaaaagaatattgattaatcaaaagcctgtgaatcctgggacatacgtttactgatatctatggtgaatagagtccaggagcagttgcataataagtacatgtaaggcctaagtttaagaattgcaattaggagtattttacatttaatttataatcttagtagaggaaaagttctgatgtgattttaaaaacagaatcccttctcgccttacttacttggtactttaaccattacaaatttattcaggaaaactaaaattatttaaagaagagacatctagttctagagtaatctggcacattcatatgtgaaaaaaattagaaatcacttgatacatctacaatacacaaatagacgtataaacattgtattttaataatactctttgtcacttcaatttaaatcattccattatgaaaatttcttaattgaagggagactatttcttcaaaactctaaattaaacagagctttatcaattaagtttacagcaatatagcctttagaaatacatatttcttcattttataataatacttcccctttaaaaatttgccatggtttgtcacagatttaaaatacaaggcacctaatgctataaaagaataatacagtaaatgtagtgtaagtgaaccagatattttctcaaatacttattctttttaaagtcccatgaaatttgcacaaacatgcttgttgcataaattaaacattttttgtgtggttaatttgcaatattctacaaaacccaaaaatataatccacacttattacaggtagcttattttagcattttacctgtcagaaatactggtctatgaacacttaagtgatttcttgaaaacattttcataatatattccagcatttaacatgtgaaaataaagtcccagaacattaggatttattccttgattagttcaaatgatttcaacagctgaattccttgagatgtgtaaggcaggttggtcctttggatggactgtagactgaaacttcctataactgtagtgatatgtacacagctacatagcaaagtgcagagattgtctcttcgctgtatagttccattatcaagctgggctacagacaacagacagctaactagctccatcctcctgagaaacactgtgcatagaaatgagactctcacactgttcgctgtcttctggaactctctgaattcgatgttttctgcatataaaagcaaatattcttctgattcccaccatcacaggatcccaattattataatggcataggagagttacaataaaaaatgaaaaaaatacagggatagctcctgcaaaaaataaccaagaaaactgcaccttttgcatacacatgtcagctattatggacagaggtattgtaaggcttagtgcaagtgtgcctatcaatgatgaggtaagaaagcagccccacaaccacaggaactctgagagtactgttccaataaggccattaatgataatgcacattaatactactttattgggaaactcgaagtcctcaaatccagtataatgaagtaaaaagaaacctggccataagagcagcagattaaacaaacctacaaaaccaaagaacattggaatatccaacttgtcttctctatctacttttctcttaatcataacaatatagacagcatagagcatggctccagcaagagaccaaatggaacctactgtgtctcttccagcaggtttttcagaccctgccaggtttaccagtacaacgcctccaatgcttaaaattacagctaatagtttagaaagggtaaatctatctccactgttacttggaaatactgcagcaaggattaaggtaaaaagtccggaagttgaagataaaatattaactatagcaacttgtgtgtctgaaagtgcttcttgatatgacaaatttgccaaaaaccacacaaagcaaaaaaaaaagctaattttcgctacttgagttgcagtaagtttccccacagttttcagtatggattcttgttctttcacaggatatgacatgcgagacaactttgcttccaatgcatgacttgacggaagctgtcgaatctccatgatattactgaacctcacacgagactttttgggggttttttcagtatcaatgtttgtgctctcaggtttttcacttggaagatcatggaatttcacaggcacatacagaggttcactcaaagaactattcatagttgtatctgttgtgcaagcagcaaagtaaccttcagcatctgcaaaaaaagcagcatgctttccgcgaagtcctcttgtacactgttgtctccatggcttccaaataataaagcccaaaaggtacaaaacaaacatagatgtttttgcaaaggtgctgaagaatggtttgttgtactgggtaaaaacatacgaagtaagttcagaggaagcaacccatatcacatcaacaagcagaagaataacaatcccaagagccattcgcctgcgctgagtgaaaccactgttctgggaattcattcggttcatgacaaatacacacaccatttgcagtcttgtcttaagagcccttctgagatcctcaagagcaatgccggaaaacttggcagatctcagtctaaaaggaggtgaagaactcagcacccctctccatccagaggaatccatccctggggacagcgtctagacactgtttctaaaagtgtcttttctgtccctgatctgctggagtggaatttggttatcggagagtaagtgatttgctgtgggtcttgaaggcacctttccaatctcttcaagtggtaaaagaaaaggattctccatgctcctccacccacctctatcaaaacatccagtcattttaaaagaaacagctgggaaaagaaatcatccttctgttttggagcggggaagacagttaaggcagcgacgcctccccggggagccgaggcgagggcgcacgcacggcttcctcaattgccagcggtgggcgcagggctccggcgcccctgtcagctcccgctccctccgcccctagagaccttcacggtttcggtcaaggcgctcctgctgccaccgagggcaggaggtggtgctgctggtgggcactccgtcccggtttgggctccggtgatgtcggggcccttccctgcctgcctacctggccttcctgccccgcgatggcgtcgtggcggcaccatgagcggaccggtcaggccccgcagccgcccagcgccacggccgcggcctcggactcacagagctgtcaccgcgcctgacatcgcgccgcactggaggcccagctcctgaagacgcggtgcccctcagggagaggctcccgacaccacccaactccactcggcccaggagggcgtggagcgggtgaggggaagggacggcacagtcagctatggccgcggaggcccggagatct

SEQ ID NO: 16192 - RNA, 6861 nt, Homo sapiens
  source 1..6861: mol_type = other RNA
gctgggattacaggcatgagcctgtgttctcccctctcttccaataatgtgtattcaacaaggccttcaggtgatgctgatgctgtctgaaagccactgctctccagcatgtggtctctgaaactttacttaggagtatgcatattaaaatatatatataacttaacactatgctactacaaagggcaaaataattcactttattgtactttattttagaataattaagacaaggataggcttcaatgaaattttgctttgatgttacatggtctgactgacactggatttcttcataagaaaaataaatgtgaaagctattccaagtaagcaaatggtggcaaaaacaatctaaagaattggttttagccaggcatggtggctcatgcctgtaatcccagcactttgggaggccagggcgggcagattacttgagctcaggagttcaagagcagcctggccaacatggtgaaaccccatctctactaaaaacacaaaaattaggcaatatagcaagaccccatctctaccaaaaatacaaaaaaactaatcaggaatgggggcacatgccagtagtcccaactactcaggagactgaggtgggaggatggcttgagcttgggaggttgcagtgagccaagatcctgccactgcactccagcctgggtgacagagtgagaccccatctcaaaaaaaaaaaaagaatttcatctcatgtcaaaaataagactcttggacagaaatcttctgcctgccttccaaggacccactgaaattaatggatactctcacatgactgactttattattaaatacttgctgtaatcacaactaggcataggaaaatcaagtagagaaatactgaatgcctagcatacaacgatctaagtgaaagttaataaaagtagctcttcagaaagacatctcatgtaaaattaaatttaaaactaaaaatttcatgaagtgacctgttaagagtttcaatttagaagctttacttttctaattttaaaatatcatgaatgaaatggtgtcttcatctaggtgcttctccatcaaaatccctagctcaaaaataaaaatcatgtttgtgtcaccccagattcaaaatgctgttattggaaatgttaccatttcacatgaacattccagtaaatatgcacatagagggtactcattacttttggttggtaatttttccttaaatatatttcaatgatttcattgtttgacattttcatagttaacgtatactgaatacagaaaattttgtaggaaaacactattttttaaatgtagtaacattaaaatattaaaatatcccgtttattaaaggctcttaagatttaaagaaaaatttcctgtgcacatacaatgtacctatgaaatactgtattattagttattgtacaggcaaatgaggctgttactataaaaaaaatgtggtgtctaaaaattgcaagtctatgtgaaaaatcaacctcaatttatctaaatgggatttgggggacacggcagactattaaaatagaactcaaacttcaaattctgtaaactgaacatctcattaatgccacttcaccatttaaaaaagtcagcacacaatgttagctatgtaagtttatctgcagatgttacaggtaattatttctgttaactcctcctaaaatattatttagtaataaagaatatttcaaaaggagagtaggtagaaacgaagatcataactatacttacttaatatgaaaatgacatttcatttatttgctaatatgtggaaaaaaattttctaattaattcctcctttatccttctttaaaaacattttatttcttcaaccagcacactgaggattagtgctatgggtattaccacagtgccctgtgaaaagacttggcttccagagaagtcataccttgcataccctggagtcatacctcaaattggctctgcatgattgattttacagcgggcattaaaattcttctgaaacaaggctgtgtacctttgagaacattcacatttaaccttgtgagctcacttctacaagaacaatgaacttatttgtcagctgccagggggaaaatcagcttaatgtaaagaattaattaaatcaggttgacagaagccaatatctcaatgtttttaaattaaaatttatttaaaggaataagtatgggtgcattacataaacctaatggttcttctaagcttcaaaaagcattcatttcaaaagtattcactttttttttttttgagacggagtctcgctgtcgcccaggctggagtgcaggggcacgatctcggctcactgcaggctccgcctcccgggttcacgccattctgctgcctcagcctcccgagcagctgggactacaggcgccgccaccacgcccggctaattctttgtatttttagtagagacggggtttcactgtgttaaccaggatggtctcgatctcctgacctcgtgatccgcccgcctcggcctcccaaagtgctgggactacaggcgtgagccaccacgcccggcccaaaagcatttactgttaaggctgcctcatttttcagctttgttgtagttgagattctgatgttcacctaacaaagtccctgacaaaacagacttccttcaatccaggtcataatttgaaacgttatacaataatgagatttaagtgatgaatggaaagaaaagaaggagactgaaaagatatcagaaatttctatttgtttttagattcagaaaaatataattacaggccaacatgggtctgacagagaggaaggacgtcagcagttacttgaatgtaaccccttcccagcatttccaaagacctgcaatgtgctcattgtgatccaagggccttgttacctagtttctaggtgatctacagaattgaaacaacccagcacaactttatttcttgagaagatgaacccttaactatgaaggtgcagaaaggaagtcttcaactgctcactcaccatggctacagtattcaaatgcaacaatcattcagataaataaaacctgtgagaaaaagcaaacaggtgggcaagcaaagcggcagtgattcatactttcagttaaccaattgaacagtggtgcttccttctgaagaagttgttcattgatttttgttttttaagaaacagaaaagcagcagtataatgaaagaagattggctgaagatctatccagcctgttaactacggcttagtacttccagaatcctgagtaacaacacatgacctgtgtgatgataagagcacagaacacatgaacaaccaaaagattctaagctcagcctctttccctatagtatttacagaataattttaaatttcagtttcacctccactacttcaacgattttaccctgtaaattgctgaaggtctttgtgaactgtcgaacagcaaaaacaaaaagtagaggtatctagattataaacttcaaccaaaagtagtccttgagtaattaaaatgttacttcattatgttctttttaaaagaaaattcctcagaagtccacattctttacatgccttcaccctgttgagctaaacaggtcaaaagtataataaactcaacattatttttaacttgcgttattggtggtgccaaatgagaaaagagctgtttttgccactttgggctggatgattaaaaaaaaaaaaaaaaaaaaagagagctgtttgtattttaaatttaatatcataaacaatttttaaaggtaatataatatagaagttctcagaatgaaacaaaaggaaggctaaacttcattttagactcatggtaacaccaaagcaattttaagaatgtgaataggaagctaaacactgcaaagagaattcttaaaaatcagattagttaagaaattttgaagagaactaaactcttcacagcaaacttgaaaagaatattgattaatcaaaagcctgtgaatcctgggacatacgtttactgatatctatggtgaatagagtccaggagcagttgcataataagtacatgtaaggcctaagtttaagaattgcaattaggagtattttacatttaatttataatcttagtagaggaaaagttctgatgtgattttaaaaacagaatcccttctcgccttacttacttggtactttaaccattacaaatttattcaggaaaactaaaattatttaaagaagagacatctagttctagagtaatctggcacattcatatgtgaaaaaaattagaaatcacttgatacatctacaatacacaaatagacgtataaacattgtattttaataatactctttgtcacttcaatttaaatcattccattatgaaaatttcttaattgaagggagactatttcttcaaaactctaaattaaacagagctttatcaattaagtttacagcaatatagcctttagaaatacatatttcttcattttataataatacttcccctttaaaaatttgccatggtttgtcacagatttaaaatacaaggcacctaatgctataaaagaataatacagtaaatgtagtgtaagtgaaccagatattttctcaaatacttattctttttaaagtcccatgaaatttgcacaaacatgcttgttgcataaattaaacattttttgtgtggttaatttgcaatattctacaaaacccaaaaatataatccacacttattacaggtagcttattttagcattttacctgtcagaaatactggtctatgaacacttaagtgatttcttgaaaacattttcataatatattccagcatttaacatgtgaaaataaagtcccagaacattaggatttattccttgattagttcaaatgatttcaacagctgaattccttgagatgtgtaaggcaggttggtcctttggatggactgtagactgaaacttcctataactgtagtgatatgtacacagctacatagcaaagtgcttcattatgaaaatgaagaaaacaggtatgagaaaaatatattttagagtttcaaagaactcaaactgttatttttcagactaggcactgaaacattttttctacaaaaacttgccagagattgtctcttcgctgtatagttccattatcaagctctgaattcgatgttttctgcatataaaagcaaatattcttctgattcccaccatcacaggatcccaattattataatggcataggagagttacaataaaaaatgaaaaaaatacagggatagctcctgcaaaaaataaccaagaaaactgcaccttttgcatacacatgtcagctattatggacagaggtattgtaaggcttagtgcaagtgtgcctatcaatgatgaggtaagaaagcagccccacaaccacaggaactctgagagtactgttccaataaggccattaatgataatgcacattaatactactttattgggaaactcgaagtcctcaaatccagtataatgaagtaaaaagaaacctggccataagagcagcagattaaacaaacctacaaaaccaaagaacattggaatatccaacttgtcttctctatctacttttctcttaatcataacaatatagacagcatagagcatggctccagcaagagaccaaatggaacctactgtgtctcttccagcaggtttttcagaccctgccaggtttaccagtacaacgcctccaatgaagttcaatattttatatccatttccttctttatcaagtcttaaaattacagctaatagtttagaaagggtaaatctatctccactgttacttggaaatactgcagcaaggattaaggtaaaaagtccggaagttgaagataaaatattaactatagcaacttgtgtgtctgaaagtgcttcttgatatgacaaatttgccaaaaaccacacaaagcaaaaaaaaaagctaattttcgctacttgagttgcagtaagtttccccacagttttcagtatggattcttgttctttcacaggatatgacatgcgagacaactttgcttccaatgcatgacttgacggaagctgtcgaatctccatgatattactgaacctcacacgagactttttgggggttttttcagtatcaatgtttgtgctctcaggtttttcacttggaagatcatggaatttcacaggcacatacagaggttcactcaaagaactattcatagttgtatctgttgtgcaagcagcaaagtaaccttcagcatctgcaaaaaaagcagcatgctttccgcgaagtcctcttgtacactgttgtctccatggcttccaaataataaagcccaaaaggtacaaaacaaacatagatgtttttgcaaaggtgctgaagaatggtttgttgtactgggtaaaaacatacgaagtaagttcagaggaagcaacccatatcacatcaacaagcagaagaataacaatcccaagagccattcgcctgcgctgagtgaaaccactgttctgggaattcattcggttcatgacaaatacacacaccatttgcagtcttgtcttaagagcccttctgagatcctcaagagcaatgccggaaaacttggcagatctcagtctaaaaggaggtgaagaactcagcacccctggccttcctgccccgcgatggcgtcgtggcggcaccatgagcggaccggtcaggccccgcagccgcccagcgccacggccgcggcctcggactcacagagctgtcaccgcgcctgacatcgcgccgcactggaggcccagctcctgaagacgcggtgcccctcagggagaggctcccgacaccacccaactccactcggcccaggagggcgtggagcgggtgaggggaagggacggcacagtcagctat

SEQ ID NO: 16193 - RNA, 6844 nt, Homo sapiens
  source 1..6844: mol_type = other RNA
gctgggattacaggcatgagcctgtgttctcccctctcttccaataatgtgtattcaacaaggccttcaggtgatgctgatgctgtctgaaagccactgctctccagcatgtggtctctgaaactttacttaggagtatgcatattaaaatatatatataacttaacactatgctactacaaagggcaaaataattcactttattgtactttattttagaataattaagacaaggataggcttcaatgaaattttgctttgatgttacatggtctgactgacactggatttcttcataagaaaaataaatgtgaaagctattccaagtaagcaaatggtggcaaaaacaatctaaagaattggttttagccaggcatggtggctcatgcctgtaatcccagcactttgggaggccagggcgggcagattacttgagctcaggagttcaagagcagcctggccaacatggtgaaaccccatctctactaaaaacacaaaaattaggcaatatagcaagaccccatctctaccaaaaatacaaaaaaactaatcaggaatgggggcacatgccagtagtcccaactactcaggagactgaggtgggaggatggcttgagcttgggaggttgcagtgagccaagatcctgccactgcactccagcctgggtgacagagtgagaccccatctcaaaaaaaaaaaaagaatttcatctcatgtcaaaaataagactcttggacagaaatcttctgcctgccttccaaggacccactgaaattaatggatactctcacatgactgactttattattaaatacttgctgtaatcacaactaggcataggaaaatcaagtagagaaatactgaatgcctagcatacaacgatctaagtgaaagttaataaaagtagctcttcagaaagacatctcatgtaaaattaaatttaaaactaaaaatttcatgaagtgacctgttaagagtttcaatttagaagctttacttttctaattttaaaatatcatgaatgaaatggtgtcttcatctaggtgcttctccatcaaaatccctagctcaaaaataaaaatcatgtttgtgtcaccccagattcaaaatgctgttattggaaatgttaccatttcacatgaacattccagtaaatatgcacatagagggtactcattacttttggttggtaatttttccttaaatatatttcaatgatttcattgtttgacattttcatagttaacgtatactgaatacagaaaattttgtaggaaaacactattttttaaatgtagtaacattaaaatattaaaatatcccgtttattaaaggctcttaagatttaaagaaaaatttcctgtgcacatacaatgtacctatgaaatactgtattattagttattgtacaggcaaatgaggctgttactataaaaaaaatgtggtgtctaaaaattgcaagtctatgtgaaaaatcaacctcaatttatctaaatgggatttgggggacacggcagactattaaaatagaactcaaacttcaaattctgtaaactgaacatctcattaatgccacttcaccatttaaaaaagtcagcacacaatgttagctatgtaagtttatctgcagatgttacaggtaattatttctgttaactcctcctaaaatattatttagtaataaagaatatttcaaaaggagagtaggtagaaacgaagatcataactatacttacttaatatgaaaatgacatttcatttatttgctaatatgtggaaaaaaattttctaattaattcctcctttatccttctttaaaaacattttatttcttcaaccagcacactgaggattagtgctatgggtattaccacagtgccctgtgaaaagacttggcttccagagaagtcataccttgcataccctggagtcatacctcaaattggctctgcatgattgattttacagcgggcattaaaattcttctgaaacaaggctgtgtacctttgagaacattcacatttaaccttgtgagctcacttctacaagaacaatgaacttatttgtcagctgccagggggaaaatcagcttaatgtaaagaattaattaaatcaggttgacagaagccaatatctcaatgtttttaaattaaaatttatttaaaggaataagtatgggtgcattacataaacctaatggttcttctaagcttcaaaaagcattcatttcaaaagtattcactttttttttttttgagacggagtctcgctgtcgcccaggctggagtgcaggggcacgatctcggctcactgcaggctccgcctcccgggttcacgccattctgctgcctcagcctcccgagcagctgggactacaggcgccgccaccacgcccggctaattctttgtatttttagtagagacggggtttcactgtgttaaccaggatggtctcgatctcctgacctcgtgatccgcccgcctcggcctcccaaagtgctgggactacaggcgtgagccaccacgcccggcccaaaagcatttactgttaaggctgcctcatttttcagctttgttgtagttgagattctgatgttcacctaacaaagtccctgacaaaacagacttccttcaatccaggtcataatttgaaacgttatacaataatgagatttaagtgatgaatggaaagaaaagaaggagactgaaaagatatcagaaatttctatttgtttttagattcagaaaaatataattacaggccaacatgggtctgacagagaggaaggacgtcagcagttacttgaatgtaaccccttcccagcatttccaaagacctgcaatgtgctcattgtgatccaagggccttgttacctagtttctaggtgatctacagaattgaaacaacccagcacaactttatttcttgagaagatgaacccttaactatgaaggtgcagaaaggaagtcttcaactgctcactcaccatggctacagtattcaaatgcaacaatcattcagataaataaaacctgtgagaaaaagcaaacaggtgggcaagcaaagcggcagtgattcatactttcagttaaccaattgaacagtggtgcttccttctgaagaagttgttcattgatttttgttttttaagaaacagaaaagcagcagtataatgaaagaagattggctgaagatctatccagcctgttaactacggcttagtacttccagaatcctgagtaacaacacatgacctgtgtgatgataagagcacagaacacatgaacaaccaaaagattctaagctcagcctctttccctatagtatttacagaataattttaaatttcagtttcacctccactacttcaacgattttaccctgtaaattgctgaaggtctttgtgaactgtcgaacagcaaaaacaaaaagtagaggtatctagattataaacttcaaccaaaagtagtccttgagtaattaaaatgttacttcattatgttctttttaaaagaaaattcctcagaagtccacattctttacatgccttcaccctgttgagctaaacaggtcaaaagtataataaactcaacattatttttaacttgcgttattggtggtgccaaatgagaaaagagctgtttttgccactttgggctggatgattaaaaaaaaaaaaaaaaaaaaagagagctgtttgtattttaaatttaatatcataaacaatttttaaaggtaatataatatagaagttctcagaatgaaacaaaaggaaggctaaacttcattttagactcatggtaacaccaaagcaattttaagaatgtgaataggaagctaaacactgcaaagagaattcttaaaaatcagattagttaagaaattttgaagagaactaaactcttcacagcaaacttgaaaagaatattgattaatcaaaagcctgtgaatcctgggacatacgtttactgatatctatggtgaatagagtccaggagcagttgcataataagtacatgtaaggcctaagtttaagaattgcaattaggagtattttacatttaatttataatcttagtagaggaaaagttctgatgtgattttaaaaacagaatcccttctcgccttacttacttggtactttaaccattacaaatttattcaggaaaactaaaattatttaaagaagagacatctagttctagagtaatctggcacattcatatgtgaaaaaaattagaaatcacttgatacatctacaatacacaaatagacgtataaacattgtattttaataatactctttgtcacttcaatttaaatcattccattatgaaaatttcttaattgaagggagactatttcttcaaaactctaaattaaacagagctttatcaattaagtttacagcaatatagcctttagaaatacatatttcttcattttataataatacttcccctttaaaaatttgccatggtttgtcacagatttaaaatacaaggcacctaatgctataaaagaataatacagtaaatgtagtgtaagtgaaccagatattttctcaaatacttattctttttaaagtcccatgaaatttgcacaaacatgcttgttgcataaattaaacattttttgtgtggttaatttgcaatattctacaaaacccaaaaatataatccacacttattacaggtagcttattttagcattttacctgtcagaaatactggtctatgaacacttaagtgatttcttgaaaacattttcataatatattccagcatttaacatgtgaaaataaagtcccagaacattaggatttattccttgattagttcaaatgatttcaacagctgaattccttgagatgtgtaaggcaggttggtcctttggatggactgtagactgaaacttcctataactgtagtgatatgtacacagctacatagcaaagtgcttcattatgaaaatgaagaaaacaggtatgagaaaaatatattttagagtttcaaagaactcaaactgttatttttcagactaggcactgaaacattttttctacaaaaacttgccagagattgtctcttcgctgtatagttccattatcaagctctgaattcgatgttttctgcatataaaagcaaatattcttctgattcccaccatcacaggatcccaattattataatggcataggagagttacaataaaaaatgaaaaaaatacagggatagctcctgcaaaaaataaccaagaaaactgcaccttttgcatacacatgtcagctattatggacagaggtattgtaaggcttagtgcaagtgtgcctatcaatgatgaggtaagaaagcagccccacaaccacaggaactctgagagtactgttccaataaggccattaatgataatgcacattaatactactttattgggaaactcgaagtcctcaaatccagtataatgaagtaaaaagaaacctggccataagagcagcagattaaacaaacctacaaaaccaaagaacattggaatatccaacttgtcttctctatctacttttctcttaatcataacaatatagacagcatagagcatggctccagcaagagaccaaatggaacctactgtgtctcttccagcaggtttttcagaccctgccaggtttaccagtacaacgcctccaatgcttaaaattacagctaatagtttagaaagggtaaatctatctccactgttacttggaaatactgcagcaaggattaaggtaaaaagtccggaagttgaagataaaatattaactatagcaacttgtgtgtctgaaagtgcttcttgatatgacaaatttgccaaaaaccacacaaagcaaaaaaaaaagctaattttcgctacttgagttgcagtaagtttccccacagttttcagtatggattcttgttctttcacaggatatgacatgcgagacaactttgcttccaatgcatgacttgacggaagctgtcgaatctccatgatattactgaacctcacacgagactttttgggggttttttcagtatcaatgtttgtgctctcaggtttttcacttggaagatcatggaatttcacaggcacatacagaggttcactcaaagaactattcatagttgtatctgttgtgcaagcagcaaagtaaccttcagcatctgcaaaaaaagcagcatgctttccgcgaagtcctcttgtacactgttgtctccatggcttccaaataataaagcccaaaaggtacaaaacaaacatagatgtttttgcaaaggtgctgaagaatggtttgttgtactgggtaaaaacatacgaagtaagttcagaggaagcaacccatatcacatcaacaagcagaagaataacaatcccaagagccattcgcctgcgctgagtgaaaccactgttctgggaattcattcggttcatgacaaatacacacaccatttgcagtcttgtcttaagagcccttctgagatcctcaagagcaatgccggaaaacttggcagatctcagtctaaaaggaggtgaagaactcagcacccctggccttcctgccccgcgatggcgtcgtggcggcaccatgagcggaccggtcaggccccgcagccgcccagcgccacggccgcggcctcggactcacagagctgtcaccgcgcctgacatcgcgccgcactggaggcccagctcctgaagacgcggtgcccctcagggagaggctcccgacaccacccaactccactcggcccaggagggcgtggagcgggtgaggggaagggacggcacagtcagctatggccgcggaggcccggagatct

SEQ ID NO: 16194 - RNA, 7176 nt, Homo sapiens
  source 1..7176: mol_type = other RNA
gctgggattacaggcatgagcctgtgttctcccctctcttccaataatgtgtattcaacaaggccttcaggtgatgctgatgctgtctgaaagccactgctctccagcatgtggtctctgaaactttacttaggagtatgcatattaaaatatatatataacttaacactatgctactacaaagggcaaaataattcactttattgtactttattttagaataattaagacaaggataggcttcaatgaaattttgctttgatgttacatggtctgactgacactggatttcttcataagaaaaataaatgtgaaagctattccaagtaagcaaatggtggcaaaaacaatctaaagaattggttttagccaggcatggtggctcatgcctgtaatcccagcactttgggaggccagggcgggcagattacttgagctcaggagttcaagagcagcctggccaacatggtgaaaccccatctctactaaaaacacaaaaattaggcaatatagcaagaccccatctctaccaaaaatacaaaaaaactaatcaggaatgggggcacatgccagtagtcccaactactcaggagactgaggtgggaggatggcttgagcttgggaggttgcagtgagccaagatcctgccactgcactccagcctgggtgacagagtgagaccccatctcaaaaaaaaaaaaagaatttcatctcatgtcaaaaataagactcttggacagaaatcttctgcctgccttccaaggacccactgaaattaatggatactctcacatgactgactttattattaaatacttgctgtaatcacaactaggcataggaaaatcaagtagagaaatactgaatgcctagcatacaacgatctaagtgaaagttaataaaagtagctcttcagaaagacatctcatgtaaaattaaatttaaaactaaaaatttcatgaagtgacctgttaagagtttcaatttagaagctttacttttctaattttaaaatatcatgaatgaaatggtgtcttcatctaggtgcttctccatcaaaatccctagctcaaaaataaaaatcatgtttgtgtcaccccagattcaaaatgctgttattggaaatgttaccatttcacatgaacattccagtaaatatgcacatagagggtactcattacttttggttggtaatttttccttaaatatatttcaatgatttcattgtttgacattttcatagttaacgtatactgaatacagaaaattttgtaggaaaacactattttttaaatgtagtaacattaaaatattaaaatatcccgtttattaaaggctcttaagatttaaagaaaaatttcctgtgcacatacaatgtacctatgaaatactgtattattagttattgtacaggcaaatgaggctgttactataaaaaaaatgtggtgtctaaaaattgcaagtctatgtgaaaaatcaacctcaatttatctaaatgggatttgggggacacggcagactattaaaatagaactcaaacttcaaattctgtaaactgaacatctcattaatgccacttcaccatttaaaaaagtcagcacacaatgttagctatgtaagtttatctgcagatgttacaggtaattatttctgttaactcctcctaaaatattatttagtaataaagaatatttcaaaaggagagtaggtagaaacgaagatcataactatacttacttaatatgaaaatgacatttcatttatttgctaatatgtggaaaaaaattttctaattaattcctcctttatccttctttaaaaacattttatttcttcaaccagcacactgaggattagtgctatgggtattaccacagtgccctgtgaaaagacttggcttccagagaagtcataccttgcataccctggagtcatacctcaaattggctctgcatgattgattttacagcgggcattaaaattcttctgaaacaaggctgtgtacctttgagaacattcacatttaaccttgtgagctcacttctacaagaacaatgaacttatttgtcagctgccagggggaaaatcagcttaatgtaaagaattaattaaatcaggttgacagaagccaatatctcaatgtttttaaattaaaatttatttaaaggaataagtatgggtgcattacataaacctaatggttcttctaagcttcaaaaagcattcatttcaaaagtattcactttttttttttttgagacggagtctcgctgtcgcccaggctggagtgcaggggcacgatctcggctcactgcaggctccgcctcccgggttcacgccattctgctgcctcagcctcccgagcagctgggactacaggcgccgccaccacgcccggctaattctttgtatttttagtagagacggggtttcactgtgttaaccaggatggtctcgatctcctgacctcgtgatccgcccgcctcggcctcccaaagtgctgggactacaggcgtgagccaccacgcccggcccaaaagcatttactgttaaggctgcctcatttttcagctttgttgtagttgagattctgatgttcacctaacaaagtccctgacaaaacagacttccttcaatccaggtcataatttgaaacgttatacaataatgagatttaagtgatgaatggaaagaaaagaaggagactgaaaagatatcagaaatttctatttgtttttagattcagaaaaatataattacaggccaacatgggtctgacagagaggaaggacgtcagcagttacttgaatgtaaccccttcccagcatttccaaagacctgcaatgtgctcattgtgatccaagggccttgttacctagtttctaggtgatctacagaattgaaacaacccagcacaactttatttcttgagaagatgaacccttaactatgaaggtgcagaaaggaagtcttcaactgctcactcaccatggctacagtattcaaatgcaacaatcattcagataaataaaacctgtgagaaaaagcaaacaggtgggcaagcaaagcggcagtgattcatactttcagttaaccaattgaacagtggtgcttccttctgaagaagttgttcattgatttttgttttttaagaaacagaaaagcagcagtataatgaaagaagattggctgaagatctatccagcctgttaactacggcttagtacttccagaatcctgagtaacaacacatgacctgtgtgatgataagagcacagaacacatgaacaaccaaaagattctaagctcagcctctttccctatagtatttacagaataattttaaatttcagtttcacctccactacttcaacgattttaccctgtaaattgctgaaggtctttgtgaactgtcgaacagcaaaaacaaaaagtagaggtatctagattataaacttcaaccaaaagtagtccttgagtaattaaaatgttacttcattatgttctttttaaaagaaaattcctcagaagtccacattctttacatgccttcaccctgttgagctaaacaggtcaaaagtataataaactcaacattatttttaacttgcgttattggtggtgccaaatgagaaaagagctgtttttgccactttgggctggatgattaaaaaaaaaaaaaaaaaaaaagagagctgtttgtattttaaatttaatatcataaacaatttttaaaggtaatataatatagaagttctcagaatgaaacaaaaggaaggctaaacttcattttagactcatggtaacaccaaagcaattttaagaatgtgaataggaagctaaacactgcaaagagaattcttaaaaatcagattagttaagaaattttgaagagaactaaactcttcacagcaaacttgaaaagaatattgattaatcaaaagcctgtgaatcctgggacatacgtttactgatatctatggtgaatagagtccaggagcagttgcataataagtacatgtaaggcctaagtttaagaattgcaattaggagtattttacatttaatttataatcttagtagaggaaaagttctgatgtgattttaaaaacagaatcccttctcgccttacttacttggtactttaaccattacaaatttattcaggaaaactaaaattatttaaagaagagacatctagttctagagtaatctggcacattcatatgtgaaaaaaattagaaatcacttgatacatctacaatacacaaatagacgtataaacattgtattttaataatactctttgtcacttcaatttaaatcattccattatgaaaatttcttaattgaagggagactatttcttcaaaactctaaattaaacagagctttatcaattaagtttacagcaatatagcctttagaaatacatatttcttcattttataataatacttcccctttaaaaatttgccatggtttgtcacagatttaaaatacaaggcacctaatgctataaaagaataatacagtaaatgtagtgtaagtgaaccagatattttctcaaatacttattctttttaaagtcccatgaaatttgcacaaacatgcttgttgcataaattaaacattttttgtgtggttaatttgcaatattctacaaaacccaaaaatataatccacacttattacaggtagcttattttagcattttacctgtcagaaatactggtctatgaacacttaagtgatttcttgaaaacattttcataatatattccagcatttaacatgtgaaaataaagtcccagaacattaggatttattccttgattagttcaaatgatttcaacagctgaattccttgagatgtgtaaggcaggttggtcctttggatggactgtagactgaaacttcctataactgtagtgatatgtacacagctacatagcaaagtgcttcattatgaaaatgaagaaaacaggtatgagaaaaatatattttagagtttcaaagaactcaaactgttatttttcagactaggcactgaaacattttttctacaaaaacttgccagagattgtctcttcgctgtatagttccattatcaagctgggctacagacaacagacagctaactagctccatcctcctgagaaacactgtgcatagaaatgagactctcacactgttcgctgtcttctggaactctctgaattcgatgttttctgcatataaaagcaaatattcttctgattcccaccatcacaggatcccaattattataatggcataggagagttacaataaaaaatgaaaaaaatacagggatagctcctgcaaaaaataaccaagaaaactgcaccttttgcatacacatgtcagctattatggacagaggtattgtaaggcttagtgcaagtgtgcctatcaatgatgaggtaagaaagcagccccacaaccacaggaactctgagagtactgttccaataaggccattaatgataatgcacattaatactactttattgggaaactcgaagtcctcaaatccagtataatgaagtaaaaagaaacctggccataagagcagcagattaaacaaacctacaaaaccaaagaacattggaatatccaacttgtcttctctatctacttttctcttaatcataacaatatagacagcatagagcatggctccagcaagagaccaaatggaacctactgtgtctcttccagcaggtttttcagaccctgccaggtttaccagtacaacgcctccaatgaagttcaatattttatatccatttccttctttatcaagtcttaaaattacagctaatagtttagaaagggtaaatctatctccactgttacttggaaatactgcagcaaggattaaggtaaaaagtccggaagttgaagataaaatattaactatagcaacttgtgtgtctgaaagtgcttcttgatatgacaaatttgccaaaaaccacacaaagcaaaaaaaaaagctaattttcgctacttgagttgcagtaagtttccccacagttttcagtatggattcttgttctttcacaggatatgacatgcgagacaactttgcttccaatgcatgacttgacggaagctgtcgaatctccatgatattactgaacctcacacgagactttttgggggttttttcagtatcaatgtttgtgctctcaggtttttcacttggaagatcatggaatttcacaggcacatacagaggttcactcaaagaactattcatagttgtatctgttgtgcaagcagcaaagtaaccttcagcatctgcaaaaaaagcagcatgctttccgcgaagtcctcttgtacactgttgtctccatggcttccaaataataaagcccaaaaggtacaaaacaaacatagatgtttttgcaaaggtgctgaagaatggtttgttgtactgggtaaaaacatacgaagtaagttcagaggaagcaacccatatcacatcaacaagcagaagaataacaatcccaagagccattcgcctgcgctgagtgaaaccactgttctgggaattcattcggttcatgacaaatacacacaccatttgcagtcttgtcttaagagcccttctgagatcctcaagagcaatgccggaaaacttggcagatctcagtctaaaaggaggtgaagaactcagcacccctctccatccagaggaatccatccctggggacagcgtctagacactgtttctaaaagtgtcttttctgtccctgatctgctggagtggaatttggttatcggagagtaagtgatttgctgtgggtcttgaaggcacctttccaatctcttcaagtggtaaaagaaaaggattctccatgctcctccacccacctctatcaaaacatccagtcattttaaaagaaacagctgggaaaagaaatcatccttctgttttggagcggggaagacagttaaggcagcgacgcctccccggggagccgaggcgagggcgcacgcacggcttcctcaattgccagcggtgggcgcagggctccggcgcccctgtcagctcccgctccctccgcccctagagaccttcacggtttcggtcaaggcgctcctgctgccaccgagggcaggaggtggtgctgctggtgggcactccgt

SEQ ID NO: 16195 - RNA, 6981 nt, Homo sapiens
  source 1..6981: mol_type = other RNA
gctgggattacaggcatgagcctgtgttctcccctctcttccaataatgtgtattcaacaaggccttcaggtgatgctgatgctgtctgaaagccactgctctccagcatgtggtctctgaaactttacttaggagtatgcatattaaaatatatatataacttaacactatgctactacaaagggcaaaataattcactttattgtactttattttagaataattaagacaaggataggcttcaatgaaattttgctttgatgttacatggtctgactgacactggatttcttcataagaaaaataaatgtgaaagctattccaagtaagcaaatggtggcaaaaacaatctaaagaattggttttagccaggcatggtggctcatgcctgtaatcccagcactttgggaggccagggcgggcagattacttgagctcaggagttcaagagcagcctggccaacatggtgaaaccccatctctactaaaaacacaaaaattaggcaatatagcaagaccccatctctaccaaaaatacaaaaaaactaatcaggaatgggggcacatgccagtagtcccaactactcaggagactgaggtgggaggatggcttgagcttgggaggttgcagtgagccaagatcctgccactgcactccagcctgggtgacagagtgagaccccatctcaaaaaaaaaaaaagaatttcatctcatgtcaaaaataagactcttggacagaaatcttctgcctgccttccaaggacccactgaaattaatggatactctcacatgactgactttattattaaatacttgctgtaatcacaactaggcataggaaaatcaagtagagaaatactgaatgcctagcatacaacgatctaagtgaaagttaataaaagtagctcttcagaaagacatctcatgtaaaattaaatttaaaactaaaaatttcatgaagtgacctgttaagagtttcaatttagaagctttacttttctaattttaaaatatcatgaatgaaatggtgtcttcatctaggtgcttctccatcaaaatccctagctcaaaaataaaaatcatgtttgtgtcaccccagattcaaaatgctgttattggaaatgttaccatttcacatgaacattccagtaaatatgcacatagagggtactcattacttttggttggtaatttttccttaaatatatttcaatgatttcattgtttgacattttcatagttaacgtatactgaatacagaaaattttgtaggaaaacactattttttaaatgtagtaacattaaaatattaaaatatcccgtttattaaaggctcttaagatttaaagaaaaatttcctgtgcacatacaatgtacctatgaaatactgtattattagttattgtacaggcaaatgaggctgttactataaaaaaaatgtggtgtctaaaaattgcaagtctatgtgaaaaatcaacctcaatttatctaaatgggatttgggggacacggcagactattaaaatagaactcaaacttcaaattctgtaaactgaacatctcattaatgccacttcaccatttaaaaaagtcagcacacaatgttagctatgtaagtttatctgcagatgttacaggtaattatttctgttaactcctcctaaaatattatttagtaataaagaatatttcaaaaggagagtaggtagaaacgaagatcataactatacttacttaatatgaaaatgacatttcatttatttgctaatatgtggaaaaaaattttctaattaattcctcctttatccttctttaaaaacattttatttcttcaaccagcacactgaggattagtgctatgggtattaccacagtgccctgtgaaaagacttggcttccagagaagtcataccttgcataccctggagtcatacctcaaattggctctgcatgattgattttacagcgggcattaaaattcttctgaaacaaggctgtgtacctttgagaacattcacatttaaccttgtgagctcacttctacaagaacaatgaacttatttgtcagctgccagggggaaaatcagcttaatgtaaagaattaattaaatcaggttgacagaagccaatatctcaatgtttttaaattaaaatttatttaaaggaataagtatgggtgcattacataaacctaatggttcttctaagcttcaaaaagcattcatttcaaaagtattcactttttttttttttgagacggagtctcgctgtcgcccaggctggagtgcaggggcacgatctcggctcactgcaggctccgcctcccgggttcacgccattctgctgcctcagcctcccgagcagctgggactacaggcgccgccaccacgcccggctaattctttgtatttttagtagagacggggtttcactgtgttaaccaggatggtctcgatctcctgacctcgtgatccgcccgcctcggcctcccaaagtgctgggactacaggcgtgagccaccacgcccggcccaaaagcatttactgttaaggctgcctcatttttcagctttgttgtagttgagattctgatgttcacctaacaaagtccctgacaaaacagacttccttcaatccaggtcataatttgaaacgttatacaataatgagatttaagtgatgaatggaaagaaaagaaggagactgaaaagatatcagaaatttctatttgtttttagattcagaaaaatataattacaggccaacatgggtctgacagagaggaaggacgtcagcagttacttgaatgtaaccccttcccagcatttccaaagacctgcaatgtgctcattgtgatccaagggccttgttacctagtttctaggtgatctacagaattgaaacaacccagcacaactttatttcttgagaagatgaacccttaactatgaaggtgcagaaaggaagtcttcaactgctcactcaccatggctacagtattcaaatgcaacaatcattcagataaataaaacctgtgagaaaaagcaaacaggtgggcaagcaaagcggcagtgattcatactttcagttaaccaattgaacagtggtgcttccttctgaagaagttgttcattgatttttgttttttaagaaacagaaaagcagcagtataatgaaagaagattggctgaagatctatccagcctgttaactacggcttagtacttccagaatcctgagtaacaacacatgacctgtgtgatgataagagcacagaacacatgaacaaccaaaagattctaagctcagcctctttccctatagtatttacagaataattttaaatttcagtttcacctccactacttcaacgattttaccctgtaaattgctgaaggtctttgtgaactgtcgaacagcaaaaacaaaaagtagaggtatctagattataaacttcaaccaaaagtagtccttgagtaattaaaatgttacttcattatgttctttttaaaagaaaattcctcagaagtccacattctttacatgccttcaccctgttgagctaaacaggtcaaaagtataataaactcaacattatttttaacttgcgttattggtggtgccaaatgagaaaagagctgtttttgccactttgggctggatgattaaaaaaaaaaaaaaaaaaaaagagagctgtttgtattttaaatttaatatcataaacaatttttaaaggtaatataatatagaagttctcagaatgaaacaaaaggaaggctaaacttcattttagactcatggtaacaccaaagcaattttaagaatgtgaataggaagctaaacactgcaaagagaattcttaaaaatcagattagttaagaaattttgaagagaactaaactcttcacagcaaacttgaaaagaatattgattaatcaaaagcctgtgaatcctgggacatacgtttactgatatctatggtgaatagagtccaggagcagttgcataataagtacatgtaaggcctaagtttaagaattgcaattaggagtattttacatttaatttataatcttagtagaggaaaagttctgatgtgattttaaaaacagaatcccttctcgccttacttacttggtactttaaccattacaaatttattcaggaaaactaaaattatttaaagaagagacatctagttctagagtaatctggcacattcatatgtgaaaaaaattagaaatcacttgatacatctacaatacacaaatagacgtataaacattgtattttaataatactctttgtcacttcaatttaaatcattccattatgaaaatttcttaattgaagggagactatttcttcaaaactctaaattaaacagagctttatcaattaagtttacagcaatatagcctttagaaatacatatttcttcattttataataatacttcccctttaaaaatttgccatggtttgtcacagatttaaaatacaaggcacctaatgctataaaagaataatacagtaaatgtagtgtaagtgaaccagatattttctcaaatacttattctttttaaagtcccatgaaatttgcacaaacatgcttgttgcataaattaaacattttttgtgtggttaatttgcaatattctacaaaacccaaaaatataatccacacttattacaggtagcttattttagcattttacctgtcagaaatactggtctatgaacacttaagtgatttcttgaaaacattttcataatatattccagcatttaacatgtgaaaataaagtcccagaacattaggatttattccttgattagttcaaatgatttcaacagctgaattccttgagatgtgtaaggcaggttggtcctttggatggactgtagactgaaacttcctataactgtagtgatatgtacacagctacatagcaaagtgcttcattatgaaaatgaagaaaacaggtatgagaaaaatatattttagagtttcaaagaactcaaactgttatttttcagactaggcactgaaacattttttctacaaaaacttgccagagattgtctcttcgctgtatagttccattatcaagctgggctacagacaacagacagctaactagctccatcctcctgagaaacactgtgcatagaaatgagactctcacactgttcgctgtcttctggaactctctgaattcgatgttttctgcatataaaagcaaatattcttctgattcccaccatcacaggatcccaattattataatggcataggagagttacaataaaaaatgaaaaaaatacagggatagctcctgcaaaaaataaccaagaaaactgcaccttttgcatacacatgtcagctattatggacagaggtattgtaaggcttagtgcaagtgtgcctatcaatgatgaggtaagaaagcagccccacaaccacaggaactctgagagtactgttccaataaggccattaatgataatgcacattaatactactttattgggaaactcgaagtcctcaaatccagtataatgaagtaaaaagaaacctggccataagagcagcagattaaacaaacctacaaaaccaaagaacattggaatatccaacttgtcttctctatctacttttctcttaatcataacaatatagacagcatagagcatggctccagcaagagaccaaatggaacctactgtgtctcttccagcaggtttttcagaccctgccaggtttaccagtacaacgcctccaatgaagttcaatattttatatccatttccttctttatcaagtcttaaaattacagctaatagtttagaaagggtaaatctatctccactgttacttggaaatactgcagcaaggattaaggtaaaaagtccggaagttgaagataaaatattaactatagcaacttgtgtgtctgaaagtgcttcttgatatgacaaatttgccaaaaaccacacaaagcaaaaaaaaaagctaattttcgctacttgagttgcagtaagtttccccacagttttcagtatggattcttgttctttcacaggatatgacatgcgagacaactttgcttccaatgcatgacttgacggaagctgtcgaatctccatgatattactgaacctcacacgagactttttgggggttttttcagtatcaatgtttgtgctctcaggtttttcacttggaagatcatggaatttcacaggcacatacagaggttcactcaaagaactattcatagttgtatctgttgtgcaagcagcaaagtaaccttcagcatctgcaaaaaaagcagcatgctttccgcgaagtcctcttgtacactgttgtctccatggcttccaaataataaagcccaaaaggtacaaaacaaacatagatgtttttgcaaaggtgctgaagaatggtttgttgtactgggtaaaaacatacgaagtaagttcagaggaagcaacccatatcacatcaacaagcagaagaataacaatcccaagagccattcgcctgcgctgagtgaaaccactgttctgggaattcattcggttcatgacaaatacacacaccatttgcagtcttgtcttaagagcccttctgagatcctcaagagcaatgccggaaaacttggcagatctcagtctaaaaggaggtgaagaactcagcacccctggccttcctgccccgcgatggcgtcgtggcggcaccatgagcggaccggtcaggccccgcagccgcccagcgccacggccgcggcctcggactcacagagctgtcaccgcgcctgacatcgcgccgcactggaggcccagctcctgaagacgcggtgcccctcagggagaggctcccgacaccacccaactccactcggcccaggagggcgtggagcgggtgaggggaagggacggcacagtcagctatggccgcggaggcccggagatct

SEQ ID NO: 16196 - RNA, 7457 nt, Homo sapiens
  source 1..7457: mol_type = other RNA
gctgggattacaggcatgagcctgtgttctcccctctcttccaataatgtgtattcaacaaggccttcaggtgatgctgatgctgtctgaaagccactgctctccagcatgtggtctctgaaactttacttaggagtatgcatattaaaatatatatataacttaacactatgctactacaaagggcaaaataattcactttattgtactttattttagaataattaagacaaggataggcttcaatgaaattttgctttgatgttacatggtctgactgacactggatttcttcataagaaaaataaatgtgaaagctattccaagtaagcaaatggtggcaaaaacaatctaaagaattggttttagccaggcatggtggctcatgcctgtaatcccagcactttgggaggccagggcgggcagattacttgagctcaggagttcaagagcagcctggccaacatggtgaaaccccatctctactaaaaacacaaaaattaggcaatatagcaagaccccatctctaccaaaaatacaaaaaaactaatcaggaatgggggcacatgccagtagtcccaactactcaggagactgaggtgggaggatggcttgagcttgggaggttgcagtgagccaagatcctgccactgcactccagcctgggtgacagagtgagaccccatctcaaaaaaaaaaaaagaatttcatctcatgtcaaaaataagactcttggacagaaatcttctgcctgccttccaaggacccactgaaattaatggatactctcacatgactgactttattattaaatacttgctgtaatcacaactaggcataggaaaatcaagtagagaaatactgaatgcctagcatacaacgatctaagtgaaagttaataaaagtagctcttcagaaagacatctcatgtaaaattaaatttaaaactaaaaatttcatgaagtgacctgttaagagtttcaatttagaagctttacttttctaattttaaaatatcatgaatgaaatggtgtcttcatctaggtgcttctccatcaaaatccctagctcaaaaataaaaatcatgtttgtgtcaccccagattcaaaatgctgttattggaaatgttaccatttcacatgaacattccagtaaatatgcacatagagggtactcattacttttggttggtaatttttccttaaatatatttcaatgatttcattgtttgacattttcatagttaacgtatactgaatacagaaaattttgtaggaaaacactattttttaaatgtagtaacattaaaatattaaaatatcccgtttattaaaggctcttaagatttaaagaaaaatttcctgtgcacatacaatgtacctatgaaatactgtattattagttattgtacaggcaaatgaggctgttactataaaaaaaatgtggtgtctaaaaattgcaagtctatgtgaaaaatcaacctcaatttatctaaatgggatttgggggacacggcagactattaaaatagaactcaaacttcaaattctgtaaactgaacatctcattaatgccacttcaccatttaaaaaagtcagcacacaatgttagctatgtaagtttatctgcagatgttacaggtaattatttctgttaactcctcctaaaatattatttagtaataaagaatatttcaaaaggagagtaggtagaaacgaagatcataactatacttacttaatatgaaaatgacatttcatttatttgctaatatgtggaaaaaaattttctaattaattcctcctttatccttctttaaaaacattttatttcttcaaccagcacactgaggattagtgctatgggtattaccacagtgccctgtgaaaagacttggcttccagagaagtcataccttgcataccctggagtcatacctcaaattggctctgcatgattgattttacagcgggcattaaaattcttctgaaacaaggctgtgtacctttgagaacattcacatttaaccttgtgagctcacttctacaagaacaatgaacttatttgtcagctgccagggggaaaatcagcttaatgtaaagaattaattaaatcaggttgacagaagccaatatctcaatgtttttaaattaaaatttatttaaaggaataagtatgggtgcattacataaacctaatggttcttctaagcttcaaaaagcattcatttcaaaagtattcactttttttttttttgagacggagtctcgctgtcgcccaggctggagtgcaggggcacgatctcggctcactgcaggctccgcctcccgggttcacgccattctgctgcctcagcctcccgagcagctgggactacaggcgccgccaccacgcccggctaattctttgtatttttagtagagacggggtttcactgtgttaaccaggatggtctcgatctcctgacctcgtgatccgcccgcctcggcctcccaaagtgctgggactacaggcgtgagccaccacgcccggcccaaaagcatttactgttaaggctgcctcatttttcagctttgttgtagttgagattctgatgttcacctaacaaagtccctgacaaaacagacttccttcaatccaggtcataatttgaaacgttatacaataatgagatttaagtgatgaatggaaagaaaagaaggagactgaaaagatatcagaaatttctatttgtttttagattcagaaaaatataattacaggccaacatgggtctgacagagaggaaggacgtcagcagttacttgaatgtaaccccttcccagcatttccaaagacctgcaatgtgctcattgtgatccaagggccttgttacctagtttctaggtgatctacagaattgaaacaacccagcacaactttatttcttgagaagatgaacccttaactatgaaggtgcagaaaggaagtcttcaactgctcactcaccatggctacagtattcaaatgcaacaatcattcagataaataaaacctgtgagaaaaagcaaacaggtgggcaagcaaagcggcagtgattcatactttcagttaaccaattgaacagtggtgcttccttctgaagaagttgttcattgatttttgttttttaagaaacagaaaagcagcagtataatgaaagaagattggctgaagatctatccagcctgttaactacggcttagtacttccagaatcctgagtaacaacacatgacctgtgtgatgataagagcacagaacacatgaacaaccaaaagattctaagctcagcctctttccctatagtatttacagaataattttaaatttcagtttcacctccactacttcaacgattttaccctgtaaattgctgaaggtctttgtgaactgtcgaacagcaaaaacaaaaagtagaggtatctagattataaacttcaaccaaaagtagtccttgagtaattaaaatgttacttcattatgttctttttaaaagaaaattcctcagaagtccacattctttacatgccttcaccctgttgagctaaacaggtcaaaagtataataaactcaacattatttttaacttgcgttattggtggtgccaaatgagaaaagagctgtttttgccactttgggctggatgattaaaaaaaaaaaaaaaaaaaaagagagctgtttgtattttaaatttaatatcataaacaatttttaaaggtaatataatatagaagttctcagaatgaaacaaaaggaaggctaaacttcattttagactcatggtaacaccaaagcaattttaagaatgtgaataggaagctaaacactgcaaagagaattcttaaaaatcagattagttaagaaattttgaagagaactaaactcttcacagcaaacttgaaaagaatattgattaatcaaaagcctgtgaatcctgggacatacgtttactgatatctatggtgaatagagtccaggagcagttgcataataagtacatgtaaggcctaagtttaagaattgcaattaggagtattttacatttaatttataatcttagtagaggaaaagttctgatgtgattttaaaaacagaatcccttctcgccttacttacttggtactttaaccattacaaatttattcaggaaaactaaaattatttaaagaagagacatctagttctagagtaatctggcacattcatatgtgaaaaaaattagaaatcacttgatacatctacaatacacaaatagacgtataaacattgtattttaataatactctttgtcacttcaatttaaatcattccattatgaaaatttcttaattgaagggagactatttcttcaaaactctaaattaaacagagctttatcaattaagtttacagcaatatagcctttagaaatacatatttcttcattttataataatacttcccctttaaaaatttgccatggtttgtcacagatttaaaatacaaggcacctaatgctataaaagaataatacagtaaatgtagtgtaagtgaaccagatattttctcaaatacttattctttttaaagtcccatgaaatttgcacaaacatgcttgttgcataaattaaacattttttgtgtggttaatttgcaatattctacaaaacccaaaaatataatccacacttattacaggtagcttattttagcattttacctgtcagaaatactggtctatgaacacttaagtgatttcttgaaaacattttcataatatattccagcatttaacatgtgaaaataaagtcccagaacattaggatttattccttgattagttcaaatgatttcaacagctgaattccttgagatgtgtaaggcaggttggtcctttggatggactgtagactgaaacttcctataactgtagtgatatgtacacagctacatagcaaagtgcttcattatgaaaatgaagaaaacaggtatgagaaaaatatattttagagtttcaaagaactcaaactgttatttttcagactaggcactgaaacattttttctacaaaaacttgccagagattgtctcttcgctgtatagttccattatcaagctgggctacagacaacagacagctaactagctccatcctcctgagaaacactgtgcatagaaatgagactctcacactgttcgctgtcttctggaactctctgaattcgatgttttctgcatataaaagcaaatattcttctgattcccaccatcacaggatcccaattattataatggcataggagagttacaataaaaaatgaaaaaaatacagggatagctcctgcaaaaaataaccaagaaaactgcaccttttgcatacacatgtcagctattatggacagaggtattgtaaggcttagtgcaagtgtgcctatcaatgatgaggtaagaaagcagccccacaaccacaggaactctgagagtactgttccaataaggccattaatgataatgcacattaatactactttattgggaaactcgaagtcctcaaatccagtataatgaagtaaaaagaaacctggccataagagcagcagattaaacaaacctacaaaaccaaagaacattggaatatccaacttgtcttctctatctacttttctcttaatcataacaatatagacagcatagagcatggctccagcaagagaccaaatggaacctactgtgtctcttccagcaggtttttcagaccctgccaggtttaccagtacaacgcctccaatgcttaaaattacagctaatagtttagaaagggtaaatctatctccactgttacttggaaatactgcagcaaggattaaggtaaaaagtccggaagttgaagataaaatattaactatagcaacttgtgtgtctgaaagtgcttcttgatatgacaaatttgccaaaaaccacacaaagcaaaaaaaaaagctaattttcgctacttgagttgcagtaagtttccccacagttttcagtatggattcttgttctttcacaggatatgacatgcgagacaactttgcttccaatgcatgacttgacggaagctgtcgaatctccatgatattactgaacctcacacgagactttttgggggttttttcagtatcaatgtttgtgctctcaggtttttcacttggaagatcatggaatttcacaggcacatacagaggttcactcaaagaactattcatagttgtatctgttgtgcaagcagcaaagtaaccttcagcatctgcaaaaaaagcagcatgctttccgcgaagtcctcttgtacactgttgtctccatggcttccaaataataaagcccaaaaggtacaaaacaaacatagatgtttttgcaaaggtgctgaagaatggtttgttgtactgggtaaaaacatacgaagtaagttcagaggaagcaacccatatcacatcaacaagcagaagaataacaatcccaagagccattcgcctgcgctgagtgaaaccactgttctgggaattcattcggttcatgacaaatacacacaccatttgcagtcttgtcttaagagcccttctgagatcctcaagagcaatgccggaaaacttggcagatctcagtctaaaaggaggtgaagaactcagcacccctctccatccagaggaatccatccctggggacagcgtctagacactgtttctaaaagtgtcttttctgtccctgatctgctggagtggaatttggttatcggagagtaagtgatttgctgtgggtcttgaaggcacctttccaatctcttcaagtggtaaaagaaaaggattctccatgctcctccacccacctctatcaaaacatccagtcattttaaaagaaacagctgggaaaagaaatcatccttctgttttggagcggggaagacagttaaggcagcgacgcctccccggggagccgaggcgagggcgcacgcacggcttcctcaattgccagcggtgggcgcagggctccggcgcccctgtcagctcccgctccctccgcccctagagaccttcacggtttcggtcaaggcgctcctgctgccaccgagggcaggaggtggtgctgctggtgggcactccgtcccggtttgggctccggtgatgtcggggcccttccctgcctgcctacctggccttcctgccccgcgatggcgtcgtggcggcaccatgagcggaccggtcaggccccgcagccgcccagcgccacggccgcggcctcggactcacagagctgtcaccgcgcctgacatcgcgccgcactggaggcccagctcctgaagacgcggtgcccctcagggagaggctcccgacaccacccaactccactcggcccaggagggcgtggagcgggtgaggggaagggacggcacagtcagctatggccgcggaggcccggagatct

SEQ ID NO: 16197 - RNA, 6942 nt, Homo sapiens
  source 1..6942: mol_type = other RNA
gctgggattacaggcatgagcctgtgttctcccctctcttccaataatgtgtattcaacaaggccttcaggtgatgctgatgctgtctgaaagccactgctctccagcatgtggtctctgaaactttacttaggagtatgcatattaaaatatatatataacttaacactatgctactacaaagggcaaaataattcactttattgtactttattttagaataattaagacaaggataggcttcaatgaaattttgctttgatgttacatggtctgactgacactggatttcttcataagaaaaataaatgtgaaagctattccaagtaagcaaatggtggcaaaaacaatctaaagaattggttttagccaggcatggtggctcatgcctgtaatcccagcactttgggaggccagggcgggcagattacttgagctcaggagttcaagagcagcctggccaacatggtgaaaccccatctctactaaaaacacaaaaattaggcaatatagcaagaccccatctctaccaaaaatacaaaaaaactaatcaggaatgggggcacatgccagtagtcccaactactcaggagactgaggtgggaggatggcttgagcttgggaggttgcagtgagccaagatcctgccactgcactccagcctgggtgacagagtgagaccccatctcaaaaaaaaaaaaagaatttcatctcatgtcaaaaataagactcttggacagaaatcttctgcctgccttccaaggacccactgaaattaatggatactctcacatgactgactttattattaaatacttgctgtaatcacaactaggcataggaaaatcaagtagagaaatactgaatgcctagcatacaacgatctaagtgaaagttaataaaagtagctcttcagaaagacatctcatgtaaaattaaatttaaaactaaaaatttcatgaagtgacctgttaagagtttcaatttagaagctttacttttctaattttaaaatatcatgaatgaaatggtgtcttcatctaggtgcttctccatcaaaatccctagctcaaaaataaaaatcatgtttgtgtcaccccagattcaaaatgctgttattggaaatgttaccatttcacatgaacattccagtaaatatgcacatagagggtactcattacttttggttggtaatttttccttaaatatatttcaatgatttcattgtttgacattttcatagttaacgtatactgaatacagaaaattttgtaggaaaacactattttttaaatgtagtaacattaaaatattaaaatatcccgtttattaaaggctcttaagatttaaagaaaaatttcctgtgcacatacaatgtacctatgaaatactgtattattagttattgtacaggcaaatgaggctgttactataaaaaaaatgtggtgtctaaaaattgcaagtctatgtgaaaaatcaacctcaatttatctaaatgggatttgggggacacggcagactattaaaatagaactcaaacttcaaattctgtaaactgaacatctcattaatgccacttcaccatttaaaaaagtcagcacacaatgttagctatgtaagtttatctgcagatgttacaggtaattatttctgttaactcctcctaaaatattatttagtaataaagaatatttcaaaaggagagtaggtagaaacgaagatcataactatacttacttaatatgaaaatgacatttcatttatttgctaatatgtggaaaaaaattttctaattaattcctcctttatccttctttaaaaacattttatttcttcaaccagcacactgaggattagtgctatgggtattaccacagtgccctgtgaaaagacttggcttccagagaagtcataccttgcataccctggagtcatacctcaaattggctctgcatgattgattttacagcgggcattaaaattcttctgaaacaaggctgtgtacctttgagaacattcacatttaaccttgtgagctcacttctacaagaacaatgaacttatttgtcagctgccagggggaaaatcagcttaatgtaaagaattaattaaatcaggttgacagaagccaatatctcaatgtttttaaattaaaatttatttaaaggaataagtatgggtgcattacataaacctaatggttcttctaagcttcaaaaagcattcatttcaaaagtattcactttttttttttttgagacggagtctcgctgtcgcccaggctggagtgcaggggcacgatctcggctcactgcaggctccgcctcccgggttcacgccattctgctgcctcagcctcccgagcagctgggactacaggcgccgccaccacgcccggctaattctttgtatttttagtagagacggggtttcactgtgttaaccaggatggtctcgatctcctgacctcgtgatccgcccgcctcggcctcccaaagtgctgggactacaggcgtgagccaccacgcccggcccaaaagcatttactgttaaggctgcctcatttttcagctttgttgtagttgagattctgatgttcacctaacaaagtccctgacaaaacagacttccttcaatccaggtcataatttgaaacgttatacaataatgagatttaagtgatgaatggaaagaaaagaaggagactgaaaagatatcagaaatttctatttgtttttagattcagaaaaatataattacaggccaacatgggtctgacagagaggaaggacgtcagcagttacttgaatgtaaccccttcccagcatttccaaagacctgcaatgtgctcattgtgatccaagggccttgttacctagtttctaggtgatctacagaattgaaacaacccagcacaactttatttcttgagaagatgaacccttaactatgaaggtgcagaaaggaagtcttcaactgctcactcaccatggctacagtattcaaatgcaacaatcattcagataaataaaacctgtgagaaaaagcaaacaggtgggcaagcaaagcggcagtgattcatactttcagttaaccaattgaacagtggtgcttccttctgaagaagttgttcattgatttttgttttttaagaaacagaaaagcagcagtataatgaaagaagattggctgaagatctatccagcctgttaactacggcttagtacttccagaatcctgagtaacaacacatgacctgtgtgatgataagagcacagaacacatgaacaaccaaaagattctaagctcagcctctttccctatagtatttacagaataattttaaatttcagtttcacctccactacttcaacgattttaccctgtaaattgctgaaggtctttgtgaactgtcgaacagcaaaaacaaaaagtagaggtatctagattataaacttcaaccaaaagtagtccttgagtaattaaaatgttacttcattatgttctttttaaaagaaaattcctcagaagtccacattctttacatgccttcaccctgttgagctaaacaggtcaaaagtataataaactcaacattatttttaacttgcgttattggtggtgccaaatgagaaaagagctgtttttgccactttgggctggatgattaaaaaaaaaaaaaaaaaaaaagagagctgtttgtattttaaatttaatatcataaacaatttttaaaggtaatataatatagaagttctcagaatgaaacaaaaggaaggctaaacttcattttagactcatggtaacaccaaagcaattttaagaatgtgaataggaagctaaacactgcaaagagaattcttaaaaatcagattagttaagaaattttgaagagaactaaactcttcacagcaaacttgaaaagaatattgattaatcaaaagcctgtgaatcctgggacatacgtttactgatatctatggtgaatagagtccaggagcagttgcataataagtacatgtaaggcctaagtttaagaattgcaattaggagtattttacatttaatttataatcttagtagaggaaaagttctgatgtgattttaaaaacagaatcccttctcgccttacttacttggtactttaaccattacaaatttattcaggaaaactaaaattatttaaagaagagacatctagttctagagtaatctggcacattcatatgtgaaaaaaattagaaatcacttgatacatctacaatacacaaatagacgtataaacattgtattttaataatactctttgtcacttcaatttaaatcattccattatgaaaatttcttaattgaagggagactatttcttcaaaactctaaattaaacagagctttatcaattaagtttacagcaatatagcctttagaaatacatatttcttcattttataataatacttcccctttaaaaatttgccatggtttgtcacagatttaaaatacaaggcacctaatgctataaaagaataatacagtaaatgtagtgtaagtgaaccagatattttctcaaatacttattctttttaaagtcccatgaaatttgcacaaacatgcttgttgcataaattaaacattttttgtgtggttaatttgcaatattctacaaaacccaaaaatataatccacacttattacaggtagcttattttagcattttacctgtcagaaatactggtctatgaacacttaagtgatttcttgaaaacattttcataatatattccagcatttaacatgtgaaaataaagtcccagaacattaggatttattccttgattagttcaaatgatttcaacagctgaattccttgagatgtgtaaggcaggttggtcctttggatggactgtagactgaaacttcctataactgtagtgatatgtacacagctacatagcaaagtgcttcattatgaaaatgaagaaaacaggtatgagaaaaatatattttagagtttcaaagaactcaaactgttatttttcagactaggcactgaaacattttttctacaaaaacttgccagagattgtctcttcgctgtatagttccattatcaagctgggctacagacaacagacagctaactagctccatcctcctgagaaacactgtgcatagaaatgagactctcacactgttcgctgtcttctggaactctctgaattcgatgttttctgcatataaaagcaaatattcttctgattcccaccatcacaggatcccaattattataatggcataggagagttacaataaaaaatgaaaaaaatacagggatagctcctgcaaaaaataaccaagaaaactgcaccttttgcatacacatgtcagctattatggacagaggtattgtaaggcttagtgcaagtgtgcctatcaatgatgaggtaagaaagcagccccacaaccacaggaactctgagagtactgttccaataaggccattaatgataatgcacattaatactactttattgggaaactcgaagtcctcaaatccagtataatgaagtaaaaagaaacctggccataagagcagcagattaaacaaacctacaaaaccaaagaacattggaatatccaacttgtcttctctatctacttttctcttaatcataacaatatagacagcatagagcatggctccagcaagagaccaaatggaacctactgtgtctcttccagcaggtttttcagaccctgccaggtttaccagtacaacgcctccaatgcttaaaattacagctaatagtttagaaagggtaaatctatctccactgttacttggaaatactgcagcaaggattaaggtaaaaagtccggaagttgaagataaaatattaactatagcaacttgtgtgtctgaaagtgcttcttgatatgacaaatttgccaaaaaccacacaaagcaaaaaaaaaagctaattttcgctacttgagttgcagtaagtttccccacagttttcagtatggattcttgttctttcacaggatatgacatgcgagacaactttgcttccaatgcatgacttgacggaagctgtcgaatctccatgatattactgaacctcacacgagactttttgggggttttttcagtatcaatgtttgtgctctcaggtttttcacttggaagatcatggaatttcacaggcacatacagaggttcactcaaagaactattcatagttgtatctgttgtgcaagcagcaaagtaaccttcagcatctgcaaaaaaagcagcatgctttccgcgaagtcctcttgtacactgttgtctccatggcttccaaataataaagcccaaaaggtacaaaacaaacatagatgtttttgcaaaggtgctgaagaatggtttgttgtactgggtaaaaacatacgaagtaagttcagaggaagcaacccatatcacatcaacaagcagaagaataacaatcccaagagccattcgcctgcgctgagtgaaaccactgttctgggaattcattcggttcatgacaaatacacacaccatttgcagtcttgtcttaagagcccttctgagatcctcaagagcaatgccggaaaacttggcagatctcagtctaaaaggaggtgaagaactcagcacccctggccttcctgccccgcgatggcgtcgtggcggcaccatgagcggaccggtcaggccccgcagccgcccagcgccacggccgcggcctcggactcacagagctgtcaccgcgcctgacatcgcgccgcactggaggcccagctcctgaagacgcggtgcccctcagggagaggctcccgacaccacccaactccactcggcccaggagggcgtggagcgggtgaggggaagggacggcacagtcagctatggccgcggaggcccggagatct

SEQ ID NO: 16198 - RNA, 1579 nt, Homo sapiens
  source 1..1579: mol_type = other RNA
gctgggattacaggcatgagccttcccgcctggccaaaagaggccaacttgaacctgggagtgaatctcagctggcacaggctgggaccttctcccacctcccagggacggtgggatgtcaacctggccttcgtgagggaggggcagtggacagtggtattgatgctgagctggttgacattgtatttgtgctgcctagctgagcacagttgtacccccacaggggagcacctgtgggggcaagtgtggctcagtgaggcccccagggcaacagaaagaacatctgtgactgagatcagagagctggctcctaacttgctgtgtgatcttgggcaagtcactcctccagccctgggtctccatgggataagaccgactggcccctggagtcccttccagttagaatggagtctccaatctgtctgacctggagcgtcagtgttcccatctgtaaaatggaagcggtgacaccagctcttggcaccctgggactgtcggggcaggacatggggacgtgaacatgagctgtccagaggggccgtactatcggatggggacatagaggaagtgcagaagaatgtggacgacagcctgcagccaaagggtgcctccatttggtgacaggctccacactgcctgggctgtggcgagaggcctggggtctccaggatgccccgcctcttgtcctccttggcctcaggcagcacatttccagtgaggaatgcgtagcagtggaggcagactcggttgggcctgttgtcgtcgtatttcagttcggcccggtagtcggagcacctggcacacaccacatagccgcaggcccggcagtggtggcgacggcgcgtcagagcgttgaagggctcctggcagcgcatgcacatggtcaccatcttgtcccggacccactgcggtgcccggaggcccagctcctcagactgcagctcctgctcctggatgtctccctcaggcccctgggccgcagccttgaaggtttcattccgcttctcgatttggtcaatggctgcttggaaggcctgcatccaggaaatcatttcctcctgggaccgggcttgcagctccagggtgcgctgcttcccggacaccaggaaggagtggggaaactcagcatccatcagctcccgcaccttcatcccggccacatcgatgcgggtcctcacctggaactgggcgcccacctggatcaccctgggcacacagtagagcagcatgttgttgaacaagaaaaggtagcgctccatggggtcgttgcggcggaaggagatcttgaggaccgggccctcacggagcagggtgttagaggggtctactatgtcgtcctcgaggcccaggcgctggtacacctcccacaggtcctgcagccgctccatctcagtgatggctgcattggagtgctgggcagctgagaagatcatgtccagggcttctgaaaggggcagggccggagtttattccctgagaatctagggctggtggctggggcaggaggtctctgggcatcggcctggtctggggcctgggctggcagcttctggatgtactccttgagcagcagctcgta

SEQ ID NO: 16199 - RNA, 2430 nt, Homo sapiens
  source 1..2430: mol_type = other RNA
gctgggattacaggcatgagccttcccgcctggccaaaagaggccaacttgaacctgggagtgaatctcagctggcacaggctgggaccttctcccacctcccagggacggtgggatgtcaacctggccttcgtgagggaggggcagtggacagtggtattgatgctgagctggttgacattgtatttgtgctgcctagctgagcacagttgtacccccacaggggagcacctgtgggggcaagtgtggctcagtgaggcccccagggcaacagaaagaacatctgtgactgagatcagagagctggctcctaacttgctgtgtgatcttgggcaagtcactcctccagccctgggtctccatgggataagaccgactggcccctggagtcccttccagttagaatggagtctccaatctgtctgacctggagcgtcagtgttcccatctgtaaaatggaagcggtgacaccagctcttggcaccctgggactgtcggggcaggacatggggacgtgaacatgagctgtccagaggggccgtactatcggatggggacatagaggaagtgcagaagaatgtggacgacagcctgcagccaaagggtgcctccatttggtgacaggctccacactgcctgggctgtggcgagaggcctggggtctccaggatgccccgcctcttgtcctccttggcctcaggcagcacatttccagtgaggaatgcgtagcagtggaggcagactcggttgggcctgttgtcgtcgtatttcagttcggcccggtagtcggagcacctggcacacaccacatagccgcaggcccggcagtggtggcgacggcgcgtcagagcgttgaagggctcctggcagcgcatgcacatggtcaccatcttgtcccggacccactgcggtgcccggaggcccagctcctcagactgcagctcctgctcctggatgtctccctcaggcccctgggccgcagccttgaaggtttcattccgcttctcgatttggtcaatggctgcttggaaggcctgcatccaggaaatcatttcctcctgggaccgggcttgcagctccagggtgcgctgcttcccggacaccaggaaggagtggggaaactcagcatccatcagctcccgcaccttcatcccggccacatcgatgcgggtcctcacctggaactgggcgcccacctggatcaccctgggcacacagtagagcagcatgttgttgaacaagaaaaggtagcgctccatggggtcgttgcggcggaaggagatcttgaggaccgggccctcacggagcagggtgttagaggggtctactatgtcgtcctcgaggcccaggcgctggtacacctcccacaggtcctgcagccgctccatctcagtgatggctgcattggagtgctgggcagctgagaagatcatgtccagggctttctgggcatcggcctggtctggggcctgggctggcagcttctggatgtactccttgagcagcagctcgtaacgtggaattctctgcactggttccagcatgtggtgctgcagggtcaggctgcccgaagcctcgctgctctggatgcgagtgagaacctcctggaagagtggagacttgtcggtccaggtggccagcagctcagccgctcgctcaaagttcttgacatactcactgtacatcttcaggaagggggccagcttctggatcacgtcaccgatgcgggggttagctgtccagtcgtccaggcgccgctgcagctctgggaggaagaactgagaatggaactgatagatggaggagatgttggagaagatgaccctgaccacatcctctgggaaggccttgctgctgcgggctgtcttcagcagctcctggaaaaacacctggtctagcaggtggaggcgcgccacataggcctgctctgtctccagcagctcctggacgatcttcttctctggctcctgcgtccccgatcctgagagggtcacaggctggcaagatttcctccaggcttcgctggacagcttgttcttcagggagttcaggtacctcctgctgactgtcctgggctcagaccccacggcctccccgacattcgtcttctcccgtggtcctggggactcgggaggcctgcactcagggcggtgatgcacgtcctctagcctctggcctctgggtgctgcttctggggtcctgctattctcaaacacagtgaccaggttggacacagatgccagcttctcctcacttgcccccttcatcctgccggtttccggggtggatctcagctaccctcgaagcagagagagaggcctccagccagcacactcagccacgctggcctgggacagataggctaaatcacccatgaatctgttctgatctttcttgagggctcagaaggtcggctcttggcttcagagt

SEQ ID NO: 16200 - RNA, 1606 nt, Homo sapiens
  source 1..1606: mol_type = other RNA
gctgggattacaggcatgagccttcccgcctggccaaaagaggccaacttgaacctgggagtgaatctcagctggcacaggctgggaccttctcccacctcccagggacggtgggatgtcaacctggccttcgtgagggaggggcagtggacagtggtattgatgctgagctggttgacattgtatttgtgctgcctagctgagcacagttgtacccccacaggggagcacctgtgggggcaagtgtggctcagtgaggcccccagggcaacagaaagaacatctgtgactgagatcagagagctggctcctaacttgctgtgtgatcttgggcaagtcactcctccagccctgggtctccatgggataagaccgactggcccctggagtcccttccagttagaatggagtctccaatctgtctgacctggagcgtcagtgttcccatctgtaaaatggaagcggtgacaccagctcttggcaccctgggactgtcggggcaggacatggggacgtgaacatgagctgtccagaggggccgtactatcggatggggacatagaggaagtgcagaagaatgtggacgacagcctgcagccaaagggtgcctccatttggtgacaggctccacactgcctgggctgtggcgagaggcctggggtctccaggatgccccgcctcttgtcctccttggcctcaggcagcacatttccagtgaggaatgcgtagcagtggaggcagactcggttgggcctgttgtcgtcgtatttcagttcggcccggtagtcggagcacctggcacacaccactggctcagcaggcacgaagatatagccgcaggcccggcagtggtggcgacggcgcgtcagagcgttgaagggctcctggcagcgcatgcacatggtcaccatcttgtcccggacccactgcggtgcccggaggcccagctcctcagactgcagctcctgctcctggatgtctccctcaggcccctgggccgcagccttgaaggtttcattccgcttctcgatttggtcaatggctgcttggaaggcctgcatccaggaaatcatttcctcctgggaccgggcttgcagctccagggtgcgctgcttcccggacaccaggaaggagtggggaaactcagcatccatcagctcccgcaccttcatcccggccacatcgatgcgggtcctcacctggaactgggcgcccacctggatcaccctgggcacacagtagagcagcatgttgttgaacaagaaaaggtagcgctccatggggtcgttgcggcggaaggagatcttgaggaccgggccctcacggagcagggtgttagaggggtctactatgtcgtcctcgaggcccaggcgctggtacacctcccacaggtcctgcagccgctccatctcagtgatggctgcattggagtgctgggcagctgagaagatcatgtccagggcttctgaaaggggcagggccggagtttattccctgagaatctagggctggtggctggggcaggaggtctctgggcatcggcctggtctggggcctgggctggcagcttctggatgtactccttgagcagcagctcgtaacgtgg

SEQ ID NO: 16201 - RNA, 1555 nt, Homo sapiens
  source 1..1555: mol_type = other RNA
gctgggattacaggcatgagccttcccgcctggccaaaagaggccaacttgaacctgggagtgaatctcagctggcacaggctgggaccttctcccacctcccagggacggtgggatgtcaacctggccttcgtgagggaggggcagtggacagtggtattgatgctgagctggttgacattgtatttgtgctgcctagctgagcacagttgtacccccacaggggagcacctgtgggggcaagtgtggctcagtgaggcccccagggcaacagaaagaacatctgtgactgagatcagagagctggctcctaacttgctgtgtgatcttgggcaagtcactcctccagccctgggtctccatgggataagaccgactggcccctggagtcccttccagttagaatggagtctccaatctgtctgacctggagcgtcagtgttcccatctgtaaaatggaagcggtgacaccagctcttggcaccctgggactgtcggggcaggacatggggacgtgaacatgagctgtccagaggggccgtactatcggatggggacatagaggaagtgcagaagaatgtggacgacagcctgcagccaaagggtgcctccatttggtgacaggctccacactgcctgggctgtggcgagaggcctggggtctccaggatgccccgcctcttgtcctccttggcctcaggcagcacatttccagtgaggaatgcgtagcagtggaggcagactcggttgggcctgttgtcgtcgtatttcagttcggcccggtagtcggagcacctggcacacaccactggctcagcaggcacgaagatatagccgcaggcccggcagtggtggcgacggcgcgtcagagcgttgaagggctcctggcagcgcatgcacatggtcaccatcttgtcccggacccactgcggtgcccggaggcccagctcctcagactgcagctcctgctcctggatgtctccctcaggcccctgggccgcagccttgaaggtttcattccgcttctcgatttggtcaatggctgcttggaaggcctgcatccaggaaatcatttcctcctgggaccgggcttgcagctccagggtgcgctgcttcccggacaccaggaaggagtggggaaactcagcatccatcagctcccgcaccttcatcccggccacatcgatgcgggtcctcacctggaactgggcgcccacctggatcaccctgggcacacagtagagcagcatgttgttgaacaagaaaaggtagcgctccatggggtcgttgcggcggaaggagatcttgaggaccgggccctcacggagcagggtgttagaggggtctactatgtcgtcctcgaggcccaggcgctggtacacctcccacaggtcctgcagccgctccatctcagtgatggctgcattggagtgctgggcagctgagaagatcatgtccagggcttctggatgcgagtgagaacctcctggaagagtggagacttgtcggtccaggtggccagcagctcagccgctcgctcaaagttcttgacata

SEQ ID NO: 16202 - RNA, 2451 nt, Homo sapiens
  source 1..2451: mol_type = other RNA
gctgggattacaggcatgagccttcccgcctggccaaaagaggccaacttgaacctgggagtgaatctcagctggcacaggctgggaccttctcccacctcccagggacggtgggatgtcaacctggccttcgtgagggaggggcagtggacagtggtattgatgctgagctggttgacattgtatttgtgctgcctagctgagcacagttgtacccccacaggggagcacctgtgggggcaagtgtggctcagtgaggcccccagggcaacagaaagaacatctgtgactgagatcagagagctggctcctaacttgctgtgtgatcttgggcaagtcactcctccagccctgggtctccatgggataagaccgactggcccctggagtcccttccagttagaatggagtctccaatctgtctgacctggagcgtcagtgttcccatctgtaaaatggaagcggtgacaccagctcttggcaccctgggactgtcggggcaggacatggggacgtgaacatgagctgtccagaggggccgtactatcggatggggacatagaggaagtgcagaagaatgtggacgacagcctgcagccaaagggtgcctccatttggtgacaggctccacactgcctgggctgtggcgagaggcctggggtctccaggatgccccgcctcttgtcctccttggcctcaggcagcacatttccagtgaggaatgcgtagcagtggaggcagactcggttgggcctgttgtcgtcgtatttcagttcggcccggtagtcggagcacctggcacacaccactggctcagcaggcacgaagatatagccgcaggcccggcagtggtggcgacggcgcgtcagagcgttgaagggctcctggcagcgcatgcacatggtcaccatcttgtcccggacccactgcggtgcccggaggcccagctcctcagactgcagctcctgctcctggatgtctccctcaggcccctgggccgcagccttgaaggtttcattccgcttctcgatttggtcaatggctgcttggaaggcctgcatccaggaaatcatttcctcctgggaccgggcttgcagctccagggtgcgctgcttcccggacaccaggaaggagtggggaaactcagcatccatcagctcccgcaccttcatcccggccacatcgatgcgggtcctcacctggaactgggcgcccacctggatcaccctgggcacacagtagagcagcatgttgttgaacaagaaaaggtagcgctccatggggtcgttgcggcggaaggagatcttgaggaccgggccctcacggagcagggtgttagaggggtctactatgtcgtcctcgaggcccaggcgctggtacacctcccacaggtcctgcagccgctccatctcagtgatggctgcattggagtgctgggcagctgagaagatcatgtccagggctttctgggcatcggcctggtctggggcctgggctggcagcttctggatgtactccttgagcagcagctcgtaacgtggaattctctgcactggttccagcatgtggtgctgcagggtcaggctgcccgaagcctcgctgctctggatgcgagtgagaacctcctggaagagtggagacttgtcggtccaggtggccagcagctcagccgctcgctcaaagttcttgacatactcactgtacatcttcaggaagggggccagcttctggatcacgtcaccgatgcgggggttagctgtccagtcgtccaggcgccgctgcagctctgggaggaagaactgagaatggaactgatagatggaggagatgttggagaagatgaccctgaccacatcctctgggaaggccttgctgctgcgggctgtcttcagcagctcctggaaaaacacctggtctagcaggtggaggcgcgccacataggcctgctctgtctccagcagctcctggacgatcttcttctctggctcctgcgtccccgatcctgagagggtcacaggctggcaagatttcctccaggcttcgctggacagcttgttcttcagggagttcaggtacctcctgctgactgtcctgggctcagaccccacggcctccccgacattcgtcttctcccgtggtcctggggactcgggaggcctgcactcagggcggtgatgcacgtcctctagcctctggcctctgggtgctgcttctggggtcctgctattctcaaacacagtgaccaggttggacacagatgccagcttctcctcacttgcccccttcatcctgccggtttccggggtggatctcagctaccctcgaagcagagagagaggcctccagccagcacactcagccacgctggcctgggacagataggctaaatcacccatgaatctgttctgatctttcttgagggctcagaaggtcggctcttggcttcagagt

SEQ ID NO: 16203 - RNA, 2283 nt, Homo sapiens
  source 1..2283: mol_type = other RNA
gctgggattacaggcatgagccttcccgcctggccaaaagaggccaacttgaacctgggagtgaatctcagctggcacaggctgggaccttctcccacctcccagggacggtgggatgtcaacctggccttcgtgagggaggggcagtggacagtggtattgatgctgagctggttgacattgtatttgtgctgcctagctgagcacagttgtacccccacaggggagcacctgtgggggcaagtgtggctcagtgaggcccccagggcaacagaaagaacatctgtgactgagatcagagagctggctcctaacttgctgtgtgatcttgggcaagtcactcctccagccctgggtctccatgggataagaccgactggcccctggagtcccttccagttagaatggagtctccaatctgtctgacctggagcgtcagtgttcccatctgtaaaatggaagcggtgacaccagctcttggcaccctgggactgtcggggcaggacatggggacgtgaacatgagctgtccagaggggccgtactatcggatggggacatagaggaagtgcagaagaatgtggacgacagcctgcagccaaagggtgcctccatttggtgacaggctccacactgcctgggctgtggcgagaggcctggggtctccaggatgccccgcctcttgtcctccttggcctcaggcagcacatttccagtgaggaatgcgtagcagtggaggcagactcggttgggcctgttgtcgtcgtatttcagttcggcccggtagtcggagcacctggcacacaccactggctcagcaggcacgaagatatagccgcaggcccggcagtggtggcgacggcgcgtcagagcgttgaagggctcctggcagcgcatgcacatggtcaccatcttgtcccggacccactgcggtgcccggaggcccagctcctcagactgcagctcctgctcctggatgtctccctcaggcccctgggccgcagccttgaaggtttcattccgcttctcgatttggtcaatggctgcttggaaggcctgcatccaggaaatcatttcctcctgggaccgggcttgcagctccagggtgcgctgcttcccggacaccaggaaggagtggggaaactcagcatccatcagctcccgcaccttcatcccggccacatcgatgcgggtcctcacctggaactgggcgcccacctggatcaccctgggcacacagtagagcagcatgttgttgaacaagaaaaggtagcgctccatggggtcgttgcggcggaaggagatcttgaggaccgggccctcacggagcagggtgttagaggggtctactatgtcgtcctcgaggcccaggcgctggtacacctcccacaggtcctgcagccgctccatctcagtgatggctgcattggagtgctgggcagctgagaagatcatgtccagggctttctgggcatcggcctggtctggggcctgggctggcagcttctggatgtactccttgagcagcagctcgtaacgtggaattctctgcactggttccagcatgtggtgctgcagggtcaggctgcccgaagcctcgctggatgcgagtgagaacctcctggaagagtggagacttgtcggtccaggtggccagcagctcagccgctcgctcaaagttcttgacatactcactgtacatcttcaggaagggggccagcttctggatcacgtcaccgatgcgggggttagctgtccagtcgtccaggcgccgctgcagctctgggaggaagaactgagaatggaactgatagatggaggagatgttggagaagatgaccctgaccacatcctctgggaaggccttgctgctgcgggctgtcttcagcagctcctggaaaaacacctggtctagcaggtggaggcgcgccacataggcctgctctgtctccagcagctcctggacgatcttcttctctggctcctgcgtccccgatcctgagagggtcacaggctggcaagatttcctccaggcttcgctggacagcttgttcttcagggagttcaggtacctcctgctgactgtcctgggctcagaccccacggcctccccgacattcgtcttctcccgtggtcctggggactcgggaggcctgcactcagggcggtgatgcacgtcctctagcctctggcctctgggtgctgcttctggggtcctgctattctcaaacacagtgaccaggttggacacagatgccagcttctcctcacttgcccccttcat

SEQ ID NO: 16204 - RNA, 2340 nt, Homo sapiens
  source 1..2340: mol_type = other RNA
gctgggattacaggcatgagccttcccgcctggccaaaagaggccaacttgaacctgggagtgaatctcagctggcacaggctgggaccttctcccacctcccagggacggtgggatgtcaacctggccttcgtgagggaggggcagtggacagtggtattgatgctgagctggttgacattgtatttgtgctgcctagctgagcacagttgtacccccacaggggagcacctgtgggggcaagtgtggctcagtgaggcccccagggcaacagaaagaacatctgtgactgagatcagagagctggctcctaacttgctgtgtgatcttgggcaagtcactcctccagccctgggtctccatgggataagaccgactggcccctggagtcccttccagttagaatggagtctccaatctgtctgacctggagcgtcagtgttcccatctgtaaaatggaagcggtgacaccagctcttggcaccctgggactgtcggggcaggacatggggacgtgaacatgagctgtccagaggggccgtactatcggatggggacatagaggaagtgcagaagaatgtggacgacagcctgcagccaaagggtgcctccatttggtgacaggctccacactgcctgggctgtggcgagaggcctggggtctccaggatgccccgcctcttgtcctccttggcctcaggcagcacatttccagtgaggaatgcgtagcagtggaggcagactcggttgggcctgttgtcgtcgtatttcagttcggcccggtagtcggagcacctggcacacaccactggctcagcaggcacgaagatatagccgcaggcccggcagtggtggcgacggcgcgtcagagcgttgaagggctcctggcagcgcatgcacatggtcaccatcttgtcccggacccactgcggtgcccggaggcccagctcctcagactgcagctcctgctcctggatgtctccctcaggcccctgggccgcagccttgaaggtttcattccgcttctcgatttggtcaatggctgcttggaaggcctgcatccaggaaatcatttcctcctgggaccgggcttgcagctccagggtgcgctgcttcccggacaccaggaaggagtggggaaactcagcatccatcagctcccgcaccttcatcccggccacatcgatgcgggtcctcacctggaactgggcgcccacctggatcaccctgggcacacagtagagcagcatgttgttgaacaagaaaaggtagcgctccatggggtcgttgcggcggaaggagatcttgaggaccgggccctcacggagcagggtgttagaggggtctactatgtcgtcctcgaggcccaggcgctggtacacctcccacaggtcctgcagccgctccatctcagtgatggctgcattggagtgctgggcagctgagaagatcatgtccagggctttctgggcatcggcctggtctggggcctgggctggcagcttctggatgtactccttgagcagcagctcgtaacgtggaattctctgcactggttccagcatgtggtgctgcagggtcaggctgcccgaagcctcgctggatgcgagtgagaacctcctggaagagtggagacttgtcggtccaggtggccagcagctcagccgctcgctcaaagttcttgacatactcactgtacatcttcaggaagggggccagcttctggatcacgtcaccgatgcgggggttagctgtcctgcaggaggggcacagggattgccctcagcctagagacctcctctcgactctagatagggccaggtgaggccaggctccctgaatcccccaaagcaaactttccacggcaattctgggtgtgggcggggtacgggggtgtcatcctcacatgcgcccctctactccttagactgtgagcctcctgaggccaaaggctgttctggtcccaggttggcctcatccacaaggcccggcacagtgttgggcccacagcaggtgttcagtaactgctcagtgcttcattatgtaacaataacgagggctacctaccaagcactacccaggacatgatgcatgtctcattccatgtaattctcacaaccctgtaggtgggggcagccactagcccatcatagaggtgaggaagtggaggctcagaggggtacgaacttctccaggattggccagccacagtggcttacacctgtactcgcagcactctgcaaggcctgaggcaggcaggcaggttgagcccaggagttcaagaccagcctgagcagcatggtgaaacctcattccatgcccctcacactgaaaaaaaat

SEQ ID NO: 16205 - RNA, 1890 nt, Homo sapiens
  source 1..1890: mol_type = other RNA
gctgggattacaggcatgagccttgatagggttgggggcagaagacaaaaaggccagagtcaggctagagggcctgaacccagggcaggattatatccaaaagcactgacccagaggggtccccagataaccccaggtttgctctcaggatagaccatgcagaaggcatggagtctgagccctgggaaagctgagaagagtgtcagtccccaggtggccctggacccaggccatttctctgtagacaatgaggaatttgggctccagtctcccatttcccctccctgctgtggaaggtcatccccatctgagagcccagaaacacttggggcggctgcattcccacctctttcagctggggctggtttgctgcaaacatttctgcaaatcctccagcactctctcaggatggaggacttgccctcgttagagtaacaggaaccaagatttgggggtcagacagagctgggttcagttccttcctcagcggcttcccagtcacatcacttcctttcttgctgagtctcctttctccttcaaagtccactcgtccatccccattgaggtccacatctcggataatttcctctatgtctcggtgtcccacctgatgacccaggagcttcctcatagcctctcgcagctcactggtgcttatttccccatcaccattggtgtcaaactctcggaaagcatctcgcagttcctttacaccaatcatatctgctgtctctgccaggagtttaggccccattagctccacgaagtcatcaaaatctacatggccacccaggttcatgttgatctgctgggacagttcgatgagctccatctcggtgggcatgtagcccatggtgcgcatgcagttgcccagatcccggcagttgatgtagccatccttgtccttgtcgaattctctgaaggcctctcggagctcttcaatttcctctggtcgcagtgatctatcaggctgcctgttctcagcgaagcccttgcgcaggaaaatgcaggcagggcccagcaggttgtgcatgactgcgcagttctgggccagcatcaggagcggtcccgggagctcggcgtcagccgccagcccctcctcgctcgtctgcaccaccatgtagctggtctgttcctcctggcacatcttcagccagcaccaagcaaatgcaaaagagaggcagggtgtcacctccctgcccagcctggctcctggtcccgggaggggctttccgcaagaggggaccctgagagtcaaggagcggggttcagagagccctgagcgtgcacaggcatcaaattggtccaacagacagagtctccaatccttgacggaaatggtggttccggggagagctgaatgtgatgccctctgtgtggcacatgcgcacacacacacacacacacacgcacgcacgcactggcacatacatatgcacagaatcacacacccaagtgcatgaagagacaggggcagcggggggcttctattctcaccaatgggaagtgttcactcagagcctaatgagacaacatcctttcccaaaatgctcccaacctcccaattcagtcaatctccagggctaagtcattcctcccagctcccaaacagacttgtcctactccagccagatccccgctggaaggcagtgagggcaatcggagctggcagcatggagaccaggcttggctggtctgccagaccagaggttgcacatgcaggtgccattgctgacataaatgaagcaggcagggtgtgagaggtggggactggggcaaagtggaaacatgccccctcctttttcgtgtgtggctagtgcactctgtcgcccaggctggagtgcagtggcgtgatcttggctcactgcaacctctgactcccggattcaa

SEQ ID NO: 16206 - RNA, 4109 nt, Homo sapiens
  source 1..4109: mol_type = other RNA
gctgggattacaggcatgagccttgatagggttgggggcagaagacaaaaaggccagagtcaggctagagggcctgaacccagggcaggattatatccaaaagcactgacccagaggggtccccagataaccccaggtttgctctcaggatagaccatgcagaaggcatggagtctgagccctgggaaagctgagaagagtgtcagtccccaggtggccctggacccaggccatttctctgtagacaatgaggaatttgggctccagtctcccatttcccctccctgctgtggaaggtcatccccatctgagagcccagaaacacttggggcggctgcattcccacctctttcagctggggctggtttgctgcaaacatttctgcaaatcctccagcactctctcaggatggaggacttgccctcgttagagtaacaggaaccaagatttgggggtcagacagagctgggttcagttccttcctcagcggcttcccagtcacatcacttcctttcttgctgagtctcctttctccttcaaagtccactcgtccatccccattgaggtccacatctcggataatttcctctatgtctcggtgtcccacctgatgacccaggagcttcctcatagcctctcgcagctcactggtgcttatttccccatcaccattggtgtcaaactctcggaaagcatctcgcagttcctttacaccaatcatatctgctgtctctgccaggagtttaggccccattagctccacgaagtcatcaaaatctacatggccacccaggttcatgttgatctgctgggacagttcgatgagctccatctcggtgggcatgtagcccatggtgcgcatgcagttgcccagatcccggcagttgatgtagccatccttgtccttgtcgaattctctgaaggcctctcggagctcttcaatttcctctggtcgcagtgatctatcaggctgcctgttctcagcgaagcccttgcgcaggaaaatgcaggcagggcccagcaggttgtgcatgactgcgcagttctgggccagcatcaggagcggtcccgggagctcggcgtcagccgccagcccctcctcgctcgtctgcaccaccatgtagctggtctgttcctcctggcacatcttccttgagagatttctcagtggatacttgacacagttgcccatcctaagttgaggcagcccctcttgggatccccgggtccatgaaggaggctcctgggggactgagggacttccgtcccagtctctgccaaccccagcctccctccgtctgtgccgttcttcctccaggacggatgtgagccctctcttgcgcgcgtgctctcttactcgtctgcctgctcctgctctccgattttttttttttttgggtggattgtgtgtgtgtttgtgtgtgggtttaactttctgggcactttcttaaggagatgaaagcagaaggggagagtgcagggcacagggaaagtcacctggagagctgatggcagaggggaaccaagctggagaaggctgccggatcatctacatcagattagcgctcagtcctgtctctggttctctccccttctctcggcccctcctttccccgctgccaaatctgcagggagatggcctcagggaggggggcccagaatggcagctgcggctgggaattaggccagcaggcccagaaagggaagctggctagtttgggttcccgaagccagggtgcctgccgcacagctcccagccttgtgtgtgtgcgcgcgcgcacacacacacacacaaacgtgcatgcacacacacacgcgcgcacaaacacacacacacatgcatgcacacacaagcgctcagggagatgaatgccccttccaaagagcagtgagctggacaagcactcactgcccctggcaattccagctgcattgagagctgcggctccagtcgagagcctgggaggtctggtgacgcctccatcatgctccatttttcacacttgccttgtcactgaaatgggacgaggctcgggggccggcagtgcagatgagccaacagtcagatcagatccttctgctctgtgtgcaatttctctgacccgaaggaaaccaggagatggccccgaggggagcatgacggaggcagcgcaggcagagagggcatgagcaaaaggtctctgaacctcctcctcctcgccccctgcctcatccacagcaaagacctctccccagcttccttggggtgccgggcagagaagaagccctttacgaagcgctcttcgaggtcccacagctggagctttttagatgactggctcttcctcgtccctccagggtcggctttgatatgaattcatctcacgcctcagatgtccggtttgagacctacagccccagccagattccccgcgtgcaagtgtccctgtttcctgcacccagctttttccagcagggggcaccagagatagactggaagcagaactcctcccaagcccattcttgcacgctagctcagttttcagcccggagagcctcctttcccaggaacttttctcccgtgtgggggggctgctcagaactcctgttaggaagatgggtgggggcgctgcccagagggtgctcactcctagggagctgggaaggaggtccctggataactcctggacctccccggtgctgctgctgacaaccacgcaatggtttaatcaggggagttactcagcagccttgtttgggccaaacctctggagggggagatggaggaggaggagcctggggggcgggtattgatgactaaagaacagaaaagagggtgatgatgcgtgtctcctggaaacagcatgaaggaagcaggcccaggcaggggtcagtggactccaatgaatgggaaggacggggaggtctggggttgagtctagctctgccagcttcttttttttttttttttagacagtgtcttgctctgttgcccaggctggagtgcagtgccgcaatctcagctcactgcaacctctgcctcctgggttgaagcgattctcctggctcagcctcccgagtagctaggattacagacgcacaacttcatgcctggctaatttttgtatttttagtagagatggggtttcaccatgttgaacaggctactcttgaactcctgacctcaggtgatccacctgccttggcctcccgaagtgctgggattacagacatgagacaccatgcccagcgctgccagcttctgactgggtggctgcctcccattcctgaacttcagtttccgccactggaaaaatggggcttttcctagcttgcttatatagcatacatgagaaagtgtaagacaccgaatagctactggatcagtaattatttaaatggaagaaagaagtatcacttgtccagtggagaaatgtcaggcaccgtgcttggctctgggaacgttgttgggggataagagaaacacagttcctgatttcaggacgcttacattctagcaggtgggcaggagatattagagctgggacacagttatctgattacatttcagataaatgctatgaagggaaaacacaaaaactctgggaatgtgagtgaggggaatctgtctgagtctaggggatcaggaaagacttgcaggcaaaatctagaaaatagaccatatgtaggttcctttgaaacaatagtgctcactagggaccccagagggaagctcaggttaaggtccaggtatgaatgggtggatatatgtaaaggccaaaacagcacagcataaagcagagattctcaatgctggctgtagactggcataactggggagcttccccagaaattctaacttaattctgtctccaatgggcactgggcattggtgttgcttagtactcccaggtaattctaacctgcagccagtgttgggaagcactgatgtagaggctaagagcttggggcggggcgtggtggctcacacctgtaatcccagcactttgggaggcataggcaggtggatcacctgaggtcaggagttcgaggccagcctggccaacgtggtgaaacgctgtctctactaaaaaaaaaaaaaaaaaaatacaaaagttagctgggcgtgg

SEQ ID NO: 16207 - RNA, 1755 nt, Homo sapiens
  source 1..1755: mol_type = other RNA
gctgggattacaggcatgagccttgatagggttgggggcagaagacaaaaaggccagagtcaggctagagggcctgaacccagggcaggattatatccaaaagcactgacccagaggggtccccagataaccccaggtttgctctcaggatagaccatgcagaaggcatggagtctgagccctgggaaagctgagaagagtgtcagtccccaggtggccctggacccaggccatttctctgtagacaatgaggaatttgggctccagtctcccatttcccctccctgctgtggaaggtcatccccatctgagagcccagaaacacttggggcggctgcattcccacctctttcagctggggctggtttgctgcaaacatttctgcaaatcctccagcactctctcaggatggaggacttgccctcgttagagtaacaggaaccaagatttgggggtcagacagagctgggttcagttccttcctcagcggcttcccagtcacatcacttcctttcttgctgagtctcctttctccttcaaagtccactcgtccatccccattgaggtccacatctcggataatttcctctatgtctcggtgtcccacctgatgacccaggagcttcctcatagcctctcgcagctcactggtgcttatttccccatcaccattggtgtcaaactctcggaaagcatctcgcagttcctttacaccaatcatatctgctgtctctgccaggagtttaggccccattagctccacgaagtcatcaaaatctacatggccacccaggttcatgttgatctgctgggacagttcgatgagctccatctcggtgggcatgtagcccatggtgcgcatgcagttgcccagatcccggcagttgatgtagccatccttgtccttgtcgaattctctgaaggcctctcggagctcttcaatttcctctggtcgcagtgatctatcctggccaaaggcggagctgagcatggggcgcagccggtggaggaacgggtccgcctcggacgcggcggctggaacggagtccccgcggccccgggctcgcagagagccccggaggccgagcgccggggacagtccccgttcctccccatcccgcccgcgggccggcggcagcggcgacgacggcgaaggtcgggacgccgcggccggcagcgcctcccggggcctgcagtgcgcctgggggagcacacgctggctcccccgcgcgccctcctctcgcggcgccggccggcacaggggcctccgcgaactggggtccccggacgactgcggcgtcgccgggcaggagccgggtagccggcggctaggcagccccgggtcccgggcagggccgtggcggggagcccggctgcccccgctcgccgccgccgccgccgccttcagcagcgacgtcttggactcgcttttggcgatgtgcgagctcatcgcggcggggcccgcgctcgcatggcccggcgggggcggcgcggtgcggcgcggcgcggggcccccggcgggcagagaacggggctcccggcgggagccaagcccgaggacgcgctggaggcgggcgccgtcccccggccgcttaaatgcggccccgtcgccgccgcccatgtgacagcgcagcctctacgcccggagcccggagctcccggcggctggcggtgcagatctgggggcgctgccggctgtccccggagagcccacccccggctccctggcggcccaggtaccgccgcgccccgccc

SEQ ID NO: 16208 - RNA, 3929 nt, Homo sapiens
  source 1..3929: mol_type = other RNA
gctgggattacaggcatgagccttgatagggttgggggcagaagacaaaaaggccagagtcaggctagagggcctgaacccagggcaggattatatccaaaagcactgacccagaggggtccccagataaccccaggtttgctctcaggatagaccatgcagaaggcatggagtctgagccctgggaaagctgagaagagtgtcagtccccaggtggccctggacccaggccatttctctgtagacaatgaggaatttgggctccagtctcccatttcccctccctgctgtggaaggtcatccccatctgagagcccagaaacacttggggcggctgcattcccacctctttcagctggggctggtttgctgcaaacatttctgcaaatcctccagcactctctcaggatggaggacttgccctcgttagagtaacaggaaccaagatttgggggtcagacagagctgggttcagttccttcctcagcggcttcccagtcacatcacttcctttcttgctgagtctcctttctccttcaaagtccactcgtccatccccattgaggtccacatctcggataatttcctctatgtctcggtgtcccacctgatgacccaggagcttcctcatagcctctcgcagctcactggtgcttatttccccatcaccattggtgtcaaactctcggaaagcatctcgcagttcctttacaccaatcatatctgctgtctctgccaggagtttaggccccattagctccacgaagtcatcaaaatctacatggccacccaggttcatgttgatctgctgggacagttcgatgagctccatctcggtgggcatgtagcccatggtgcgcatgcagttgcccagatcccggcagttgatgtagccatccttgtccttgtcgaattctctgaaggcctctcggagctcttcaatttcctctggtcgcagtgatctatccttccttgagagatttctcagtggatacttgacacagttgcccatcctaagttgaggcagcccctcttgggatccccgggtccatgaaggaggctcctgggggactgagggacttccgtcccagtctctgccaaccccagcctccctccgtctgtgccgttcttcctccaggacggatgtgagccctctcttgcgcgcgtgctctcttactcgtctgcctgctcctgctctccgattttttttttttttgggtggattgtgtgtgtgtttgtgtgtgggtttaactttctgggcactttcttaaggagatgaaagcagaaggggagagtgcagggcacagggaaagtcacctggagagctgatggcagaggggaaccaagctggagaaggctgccggatcatctacatcagattagcgctcagtcctgtctctggttctctccccttctctcggcccctcctttccccgctgccaaatctgcagggagatggcctcagggaggggggcccagaatggcagctgcggctgggaattaggccagcaggcccagaaagggaagctggctagtttgggttcccgaagccagggtgcctgccgcacagctcccagccttgtgtgtgtgcgcgcgcgcacacacacacacacaaacgtgcatgcacacacacacgcgcgcacaaacacacacacacatgcatgcacacacaagcgctcagggagatgaatgccccttccaaagagcagtgagctggacaagcactcactgcccctggcaattccagctgcattgagagctgcggctccagtcgagagcctgggaggtctggtgacgcctccatcatgctccatttttcacacttgccttgtcactgaaatgggacgaggctcgggggccggcagtgcagatgagccaacagtcagatcagatccttctgctctgtgtgcaatttctctgacccgaaggaaaccaggagatggccccgaggggagcatgacggaggcagcgcaggcagagagggcatgagcaaaaggtctctgaacctcctcctcctcgccccctgcctcatccacagcaaagacctctccccagcttccttggggtgccgggcagagaagaagccctttacgaagcgctcttcgaggtcccacagctggagctttttagatgactggctcttcctcgtccctccagggtcggctttgatatgaattcatctcacgcctcagatgtccggtttgagacctacagccccagccagattccccgcgtgcaagtgtccctgtttcctgcacccagctttttccagcagggggcaccagagatagactggaagcagaactcctcccaagcccattcttgcacgctagctcagttttcagcccggagagcctcctttcccaggaacttttctcccgtgtgggggggctgctcagaactcctgttaggaagatgggtgggggcgctgcccagagggtgctcactcctagggagctgggaaggaggtccctggataactcctggacctccccggtgctgctgctgacaaccacgcaatggtttaatcaggggagttactcagcagccttgtttgggccaaacctctggagggggagatggaggaggaggagcctggggggcgggtattgatgactaaagaacagaaaagagggtgatgatgcgtgtctcctggaaacagcatgaaggaagcaggcccaggcaggggtcagtggactccaatgaatgggaaggacggggaggtctggggttgagtctagctctgccagcttcttttttttttttttttagacagtgtcttgctctgttgcccaggctggagtgcagtgccgcaatctcagctcactgcaacctctgcctcctgggttgaagcgattctcctggctcagcctcccgagtagctaggattacagacgcacaacttcatgcctggctaatttttgtatttttagtagagatggggtttcaccatgttgaacaggctactcttgaactcctgacctcaggtgatccacctgccttggcctcccgaagtgctgggattacagacatgagacaccatgcccagcgctgccagcttctgactgggtggctgcctcccattcctgaacttcagtttccgccactggaaaaatggggcttttcctagcttgcttatatagcatacatgagaaagtgtaagacaccgaatagctactggatcagtaattatttaaatggaagaaagaagtatcacttgtccagtggagaaatgtcaggcaccgtgcttggctctgggaacgttgttgggggataagagaaacacagttcctgatttcaggacgcttacattctagcaggtgggcaggagatattagagctgggacacagttatctgattacatttcagataaatgctatgaagggaaaacacaaaaactctgggaatgtgagtgaggggaatctgtctgagtctaggggatcaggaaagacttgcaggcaaaatctagaaaatagaccatatgtaggttcctttgaaacaatagtgctcactagggaccccagagggaagctcaggttaaggtccaggtatgaatgggtggatatatgtaaaggccaaaacagcacagcataaagcagagattctcaatgctggctgtagactggcataactggggagcttccccagaaattctaacttaattctgtctccaatgggcactgggcattggtgttgcttagtactcccaggtaattctaacctgcagccagtgttgggaagcactgatgtagaggctaagagcttggggcggggcgtggtggctcacacctgtaatcccagcactttgggaggcataggcaggtggatcacctgaggtcaggagttcgaggccagcctggccaacgtggtgaaacgctgtctctactaaaaaaaaaaaaaaaaaaatacaaaagttagctgggcgtgg

SEQ ID NO: 16209 - RNA, 34 nt, Homo sapiens
  source 1..34: mol_type = other RNA
gctgggattacaggcatgagccttgtgctcggcc

SEQ ID NO: 16210 - RNA, 2624 nt, Homo sapiens
  source 1..2624: mol_type = other RNA
gctgggcagggcttctgagctccttccaacccaagggtttcctgatttttccctcccttagggagacatgggaggttggggtaaggatatgtccaagtttgcatgaattttaaatgaaagcagttttttaaagtcccaaatgttgtcaatgatcccattttttacaataaaatgttcgtgccccacccccagaggggctgctggcccagccaagcgctgggtgccggaggctgctgctgggcaatccaggctcctggctgagactagcagggacctcctcgtcccaggggtccctcttctcccagatgagcctgtctcctgggcctcatcctcattctcctctcctgatgactcccactgtcttcctcctcttcctctcctctcgggatgaggggctactgtcctaaaagcatggcctctccttttcggccagtccacctgctccttctcctggaggtggagtcaggtacaggacggaagttccagatgtcttcacagaatttccaaatgctatttcttcatttgcaatttctgttcctgccatccgcccccatgtagcctctgcccagtcttcaacccccgcctttggagtccgtggaggaaaagagcagaaacaggagcccagagaccattccagactcaccaggtatgggcgctgccgacttaatttttacaaaaccaagccaatccgtccctaggtaaatttttgtaagcaaggtgcccactaggtaggaaggctgcatttaatgctaatttactgtaaggtctagggaagtcctttccgcttctctgggcctcagtttcctcatctgccaaatagggaaatggatgagatgattgctaaggtcccttcagttccatgagtctatgaaatgtttattgctattgcttttccttcactatcctcaccttcagagctgccagcacccacctggaatgtggttccttcacttgggccatgaatggcacaggtaaccaagagcttggcctgcctgcaagctctatggtcagacaggtgagtcctggcactgggaagggcaaaagaaaagggagagaaatgccctaggttcccactccaatcaggaggaagctcctcatcagagtgggtccatgacagctcagaggctgaagtctggatgacacagggcatccggccttccaaggcctcgggatgctgggatcctaccaccctgcagccgcttggcaggtctaaggacaaaatcaccttttgaggaagtgccaggtcagttaacatcactgtgcaaatcagaaggtccagggccagatgctttggccagagacctttcaaaccaaagccatgaggcaagcaccgctcctcccttcttccctctccttccccacaatgccctccctccccccaccctcccccaaattctaaagacttttttccccaggttctcagcctggggtattaagctgctaataacacgcctacatactcaggtggttttgttcttggtctgttgcaatggttctcaggagacatttcatttgtgtctgggacatgggaatgtcctgaactaatcttgcttaagaaaaaacaaccagaacactcccctagagatgtagcctgctcaacagctctgagttcctaccctggaccacatctgtttatgctcttcaaatggaatccagccttcagatgaaccactgcaataaaccctactctctgcttgcctctagactgggatccccagggacaggacacttagggaagagcagagaggacatggcctggtcaggtaggaggaaggggatagagctggaagggcaggggctaagagggggacagttggggagaggcaggagattagaaaaagcagcttttacaaaaaccaaaaataaaaatcaaaaccattaaagatgcataaagtgacccttgcacttccgttgtctcttcttgcaaatagaggtggtgctgctagggaactgctccagcaccggtgtaagacttgagtagttgcatacaatgtgtgactccagatttggatgggctgcaggctttaccagtgtgggggcacgtagctgtacgcaggggttccttgggccctatatgttggcatggagacagggtgtgccccaatcgccgtgtgctggggtgtagtcagcagggtacctgctgacattgccatggtggtgcctgccaccatgcccatggccacaccgttggtcctcggggcggcaacaggtgctgggtagatagcagagggaatgctgttgggctggacgaccgtggtatggtggatgacatgaggctgggcagcatacaccggctgtgtgtagtaggctccctgggcatacagattctgctgggggtaggcacttctgattggatacatggccgtctgataggggttgggtgatggggagtaggggggtggagcagtgttactctgggtcggtgggaccttgtatggtgtccccgcagtatatcctggagcataactgggactattggtggggtacaggctgggattgtaggcaggggcagctgctggataggctgtggggtaacccgtgtaggccatgttcttagggttgccataaggagccccaggctgcacggggctgtaaacagggttcattgtggaagactgaggatc

SEQ ID NO: 16211 - RNA, 2967 nt, Homo sapiens
  source 1..2967: mol_type = other RNA
gctgggcagggcttctgagctccttccaacccaagggtttcctgatttttccctcccttagggagacatgggaggttggggtaaggatatgtccaagtttgcatgaattttaaatgaaagcagttttttaaagtcccaaatgttgtcaatgatcccattttttacaataaaatgttcgtgccccacccccagaggggctgctggcccagccaagcgctgggtgccggaggctgctgctgggcaatccaggctcctggctgagactagcagggacctcctcgtcccaggggtccctcttctcccagatgagcctgtctcctgggcctcatcctcattctcctctcctgatgactcccactgtcttcctcctcttcctctcctctcgggatgaggggctactgtcctaaaagcatggcctctccttttcggccagtccacctgctccttctcctggaggtggagtcaggtacaggacggaagttccagatgtcttcacagaatttccaaatgctatttcttcatttgcaatttctgttcctgccatccgcccccatgtagcctctgcccagtcttcaacccccgcctttggagtccgtggaggaaaagagcagaaacaggagcccagagaccattccagactcaccaggtatgggcgctgccgacttaatttttacaaaaccaagccaatccgtccctaggtaaatttttgtaagcaaggtgcccactaggtaggaaggctgcatttaatgctaatttactgtaaggtctagggaagtcctttccgcttctctgggcctcagtttcctcatctgccaaatagggaaatggatgagatgattgctaaggtcccttcagttccatgagtctatgaaatgtttattgctattgcttttccttcactatcctcaccttcagagctgccagcacccacctggaatgtggttccttcacttgggccatgaatggcacaggtaaccaagagcttggcctgcctgcaagctctatggtcagacaggtgagtcctggcactgggaagggcaaaagaaaagggagagaaatgccctaggttcccactccaatcaggaggaagctcctcatcagagtgggtccatgacagctcagaggctgaagtctggatgacacagggcatccggccttccaaggcctcgggatgctgggatcctaccaccctgcagccgcttggcaggtctaaggacaaaatcaccttttgaggaagtgccaggtcagttaacatcactgtgcaaatcagaaggtccagggccagatgctttggccagagacctttcaaaccaaagccatgaggcaagcaccgctcctcccttcttccctctccttccccacaatgccctccctccccccaccctcccccaaattctaaagacttttttccccaggttctcagcctggggtattaagctgctaataacacgcctacatactcaggtggttttgttcttggtctgttgcaatggttctcaggagacatttcatttgtgtctgggacatgggaatgtcctgaactaatcttgcttaagaaaaaacaaccagaacactcccctagagatgtagcctgctcaacagctctgagttcctaccctggaccacatctgtttatgctcttcaaatggaatccagccttcagatgaaccactgcaataaaccctactctctgcttgcctctagactgggatccccagggacaggacacttagggaagagcagagaggacatggcctggtcaggtaggaggaaggggatagagctggaagggcaggggctaagagggggacagttggggagaggcaggagattagaaaaagcagcttttacaaaaaccaaaaataaaaatcaaaaccattaaagatgcataaagtgacccttgcacttccgttgtctcttcttgcaaatagaggtggtgctgctagggaactgctccagcaccggtgtaagacttgagtagttgcatacaatgtgtgactccagatttggatgggctgcaggctttaccagtgtgggggcacgtagctgtacgcaggggttccttgggccctatatgttggcatggagacagggtgtgccccaatcgccgtgtgctggggtgtagtcagcagggtacctgctgacattgccatggtggtgcctgccaccatgcccatggccacaccgttggtcctcggggcggcaacaggtgctgggtagatagcagagggaatgctgttgggctggacgaccgtggtatggtggatgacatgaggctgggcagcatacaccggctgtgtgtagtaggctccctgggcatacagattctgctgggggtaggcacttctgattggatacatggccgtctgataggggttgggtgatggggagtaggggggtggagcagtgttactctgggtcggtgggaccttgtatggtgtccccgcagtatatctgaaagccgcagaggatgcttggtaagttcggttctcggtcccggtgtccactgggaggtggaaggtgccttcagtgccacaggaagacgagttctgtggccaggcctgtttcatcagcagagttgcataagctgaatgcaggaactgaaactctggagcataactgggactattggtggggtacaggctgggattgtaggcaggggcagctgctggataggctgtggggtaacccgtgtaggccatgttcttagggttgccataaggagccccaggctgcacggggctgtaaacagggttcattgtggaagactgaggatccggtgagcagctgcaggcgaaaacggcggcggcggcggctgaggcggcgatgcccttgtcttctccggaggctacggcggcgacgctctcgcccgtgtccagtagggtggcggatggcgcgcggggaccggagcctcctcctcagcgactcggctctgaatcctctgcagtagccgccgaggagcccgac

SEQ ID NO: 16212 - RNA, 2940 nt, Homo sapiens
  source 1..2940: mol_type = other RNA
gctgggcagggcttctgagctccttccaacccaagggtttcctgatttttccctcccttagggagacatgggaggttggggtaaggatatgtccaagtttgcatgaattttaaatgaaagcagttttttaaagtcccaaatgttgtcaatgatcccattttttacaataaaatgttcgtgccccacccccagaggggctgctggcccagccaagcgctgggtgccggaggctgctgctgggcaatccaggctcctggctgagactagcagggacctcctcgtcccaggggtccctcttctcccagatgagcctgtctcctgggcctcatcctcattctcctctcctgatgactcccactgtcttcctcctcttcctctcctctcgggatgaggggctactgtcctaaaagcatggcctctccttttcggccagtccacctgctccttctcctggaggtggagtcaggtacaggacggaagttccagatgtcttcacagaatttccaaatgctatttcttcatttgcaatttctgttcctgccatccgcccccatgtagcctctgcccagtcttcaacccccgcctttggagtccgtggaggaaaagagcagaaacaggagcccagagaccattccagactcaccaggtatgggcgctgccgacttaatttttacaaaaccaagccaatccgtccctaggtaaatttttgtaagcaaggtgcccactaggtaggaaggctgcatttaatgctaatttactgtaaggtctagggaagtcctttccgcttctctgggcctcagtttcctcatctgccaaatagggaaatggatgagatgattgctaaggtcccttcagttccatgagtctatgaaatgtttattgctattgcttttccttcactatcctcaccttcagagctgccagcacccacctggaatgtggttccttcacttgggccatgaatggcacaggtaaccaagagcttggcctgcctgcaagctctatggtcagacaggtgagtcctggcactgggaagggcaaaagaaaagggagagaaatgccctaggttcccactccaatcaggaggaagctcctcatcagagtgggtccatgacagctcagaggctgaagtctggatgacacagggcatccggccttccaaggcctcgggatgctgggatcctaccaccctgcagccgcttggcaggtctaaggacaaaatcaccttttgaggaagtgccaggtcagttaacatcactgtgcaaatcagaaggtccagggccagatgctttggccagagacctttcaaaccaaagccatgaggcaagcaccgctcctcccttcttccctctccttccccacaatgccctccctccccccaccctcccccaaattctaaagacttttttccccaggttctcagcctggggtattaagctgctaataacacgcctacatactcaggtggttttgttcttggtctgttgcaatggttctcaggagacatttcatttgtgtctgggacatgggaatgtcctgaactaatcttgcttaagaaaaaacaaccagaacactcccctagagatgtagcctgctcaacagctctgagttcctaccctggaccacatctgtttatgctcttcaaatggaatccagccttcagatgaaccactgcaataaaccctactctctgcttgcctctagactgggatccccagggacaggacacttagggaagagcagagaggacatggcctggtcaggtaggaggaaggggatagagctggaagggcaggggctaagagggggacagttggggagaggcaggagattagaaaaagcagcttttacaaaaaccaaaaataaaaatcaaaaccattaaagatgcataaagtgacccttgcacttccgttgtctcttcttgcaaatagaggtggtgctgctagggaactgctccagcaccggtgtaagacttgagtagttgcatacaatgtgtgactccagatttggatgggctgcaggctttaccagtgtgggggcacgtagctgtacgcaggggttccttgggccctatatgttggcatggagacagggtgtgccccaatcgccgtgtgctggggtgtagtcagcagggtacctgctgacattgccatggtggtgcctgccaccatgcccatggccacaccgttggtcctcggggcggcaacaggtgctgggtagatagcagagggaatgctgttgggctggacgaccgtggtatggtggatgacatgaggctgggcagcatacaccggctgtgtgtagtaggctccctgggcatacagattctgctgggggtaggcacttctgattggatacatggccgtctgataggggttgggtgatggggagtaggggggtggagcagtgttactctgggtcggtgggaccttgtatggtgtccccgcagtatatctgaaagccgcagaggatgcttggtaagttcggttctcggtcccggtgtccactgggaggtggaaggtgccttcagtgccacaggaagacgagttctgtggccaggcctgtttcatcagcagagttgctggagcataactgggactattggtggggtacaggctgggattgtaggcaggggcagctgctggataggctgtggggtaacccgtgtaggccatgttcttagggttgccataaggagccccaggctgcacggggctgtaaacagggttcattgtggaagactgaggatccggtgagcagctgcaggcgaaaacggcggcggcggcggctgaggcggcgatgcccttgtcttctccggaggctacggcggcgacgctctcgcccgtgtccagtagggtggcggatggcgcgcggggaccggagcctcctcctcagcgactcggctctgaatcctctgcagtagccgccgaggagcccgac

SEQ ID NO: 16213 - RNA, 2459 nt, Homo sapiens
  source 1..2459: mol_type = other RNA
gctgggcagggcttctgagctccttccaacccaagggtttcctgatttttccctcccttagggagacatgggaggttggggtaaggatatgtccaagtttgcatgaattttaaatgaaagcagttttttaaagtcccaaatgttgtcaatgatcccattttttacaataaaatgttcgtgccccacccccagaggggctgctggcccagccaagcgctgggtgccggaggctgctgctgggcaatccaggctcctggctgagactagcagggacctcctcgtcccaggggtccctcttctcccagatgagcctgtctcctgggcctcatcctcattctcctctcctgatgactcccactgtcttcctcctcttcctctcctctcgggatgaggggctactgtcctaaaagcatggcctctccttttcggccagtccacctgctccttctcctggaggtggagtcaggtacaggacggaagttccagatgtcttcacagaatttccaaatgctatttcttcatttgcaatttctgttcctgccatccgcccccatgtagcctctgcccagtcttcaacccccgcctttggagtccgtggaggaaaagagcagaaacaggagcccagagaccattccagactcaccaggtatgggcgctgccgacttaatttttacaaaaccaagccaatccgtccctaggtaaatttttgtaagcaaggtgcccactaggtaggaaggctgcatttaatgctaatttactgtaaggtctagggaagtcctttccgcttctctgggcctcagtttcctcatctgccaaatagggaaatggatgagatgattgctaaggtcccttcagttccatgagtctatgaaatgtttattgctattgcttttccttcactatcctcaccttcagagctgccagcacccacctggaatgtggttccttcacttgggccatgaatggcacaggtaaccaagagcttggcctgcctgcaagctctatggtcagacaggtgagtcctggcactgggaagggcaaaagaaaagggagagaaatgccctaggttcccactccaatcaggaggaagctcctcatcagagtgggtccatgacagctcagaggctgaagtctggatgacacagggcatccggccttccaaggcctcgggatgctgggatcctaccaccctgcagccgcttggcaggtctaaggacaaaatcaccttttgaggaagtgccaggtcagttaacatcactgtgcaaatcagaaggtccagggccagatgctttggccagagacctttcaaaccaaagccatgaggcaagcaccgctcctcccttcttccctctccttccccacaatgccctccctccccccaccctcccccaaattctaaagacttttttccccaggttctcagcctggggtattaagctgctaataacacgcctacatactcaggtggttttgttcttggtctgttgcaatggttctcaggagacatttcatttgtgtctgggacatgggaatgtcctgaactaatcttgcttaagaaaaaacaaccagaacactcccctagagatgtagcctgctcaacagctctgagttcctaccctggaccacatctgtttatgctcttcaaatggaatccagccttcagatgaaccactgcaataaaccctactctctgcttgcctctagactgggatccccagggacaggacacttagggaagagcagagaggacatggcctggtcaggtaggaggaaggggatagagctggaagggcaggggctaagagggggacagttggggagaggcaggagattagaaaaagcagcttttacaaaaaccaaaaataaaaatcaaaaccattaaagatgcataaagtgacccttgcacttccgttgtctcttcttgcaaatagaggtggtgctgctagggaactgctccagcaccggtgtaagacttgagtagttgcatacaatgtgtgactccagatttggatgggctgcaggctttaccagtgtgggggcacgtagctgtacgcaggggttccttgggccctatatgttggcatggagacagggtgtgccccaatcgccgtgtgctggggtgtagtcagcagggtactgaaagccgcagaggatgcttggtaagttcggttctcggtcccggtgtccactgggaggtggaaggtgccttcagtgccacaggaagacgagttctgtggccaggcctgtttcatcagcagagttgcataagctgaatgcaggaactgaaactctggagcataactgggactattggtggggtacaggctgggattgtaggcaggggcagctgctggataggctgtggggtaacccgtgtaggccatgttcttagggttgccataaggagccccaggctgcacggggctgtaaacagggttcattgtggaagactgaggatc

SEQ ID NO: 16214 - RNA, 2622 nt, Homo sapiens
  source 1..2622: mol_type = other RNA
gctgggcagggcttctgagctccttccaacccaagggtttcctgatttttccctcccttagggagacatgggaggttggggtaaggatatgtccaagtttgcatgaattttaaatgaaagcagttttttaaagtcccaaatgttgtcaatgatcccattttttacaataaaatgttcgtgccccacccccagaggggctgctggcccagccaagcgctgggtgccggaggctgctgctgggcaatccaggctcctggctgagactagcagggacctcctcgtcccaggggtccctcttctcccagatgagcctgtctcctgggcctcatcctcattctcctctcctgatgactcccactgtcttcctcctcttcctctcctctcgggatgaggggctactgtcctaaaagcatggcctctccttttcggccagtccacctgctccttctcctggaggtggagtcaggtacaggacggaagttccagatgtcttcacagaatttccaaatgctatttcttcatttgcaatttctgttcctgccatccgcccccatgtagcctctgcccagtcttcaacccccgcctttggagtccgtggaggaaaagagcagaaacaggagcccagagaccattccagactcaccaggtatgggcgctgccgacttaatttttacaaaaccaagccaatccgtccctaggtaaatttttgtaagcaaggtgcccactaggtaggaaggctgcatttaatgctaatttactgtaaggtctagggaagtcctttccgcttctctgggcctcagtttcctcatctgccaaatagggaaatggatgagatgattgctaaggtcccttcagttccatgagtctatgaaatgtttattgctattgcttttccttcactatcctcaccttcagagctgccagcacccacctggaatgtggttccttcacttgggccatgaatggcacaggtaaccaagagcttggcctgcctgcaagctctatggtcagacaggtgagtcctggcactgggaagggcaaaagaaaagggagagaaatgccctaggttcccactccaatcaggaggaagctcctcatcagagtgggtccatgacagctcagaggctgaagtctggatgacacagggcatccggccttccaaggcctcgggatgctgggatcctaccaccctgcagccgcttggcaggtctaaggacaaaatcaccttttgaggaagtgccaggtcagttaacatcactgtgcaaatcagaaggtccagggccagatgctttggccagagacctttcaaaccaaagccatgaggcaagcaccgctcctcccttcttccctctccttccccacaatgccctccctccccccaccctcccccaaattctaaagacttttttccccaggttctcagcctggggtattaagctgctaataacacgcctacatactcaggtggttttgttcttggtctgttgcaatggttctcaggagacatttcatttgtgtctgggacatgggaatgtcctgaactaatcttgcttaagaaaaaacaaccagaacactcccctagagatgtagcctgctcaacagctctgagttcctaccctggaccacatctgtttatgctcttcaaatggaatccagccttcagatgaaccactgcaataaaccctactctctgcttgcctctagactgggatccccagggacaggacacttagggaagagcagagaggacatggcctggtcaggtaggaggaaggggatagagctggaagggcaggggctaagagggggacagttggggagaggcaggagattagaaaaagcagcttttacaaaaaccaaaaataaaaatcaaaaccattaaagatgcataaagtgacccttgcacttccgttgtctcttcttgcaaatagaggtggtgctgctagggaactgctccagcaccggtgtaagacttgagtagttgcatacaatgtgtgactccagatttggatgggctgcaggctttaccagtgtgggggcacgtagctgtacgcaggggttccttgggccctatatgttggcatggagacagggtgtgccccaatcgccgtgtgctggggtgtagtcagcagggtactgaaagccgcagaggatgcttggtaagttcggttctcggtcccggtgtccactgggaggtggaaggtgccttcagtgccacaggaagacgagttctgtggccaggcctgtttcatcagcagagttgctggagcataactgggactattggtggggtacaggctgggattgtaggcaggggcagctgctggataggctgtggggtaacccgtgtaggccatgttcttagggttgccataaggagccccaggctgcacggggctgtaaacagggttcattgtggaagactgaggatccggtgagcagctgcaggcgaaaacggcggcggcggcggctgaggcggcgatgcccttgtcttctccggaggctacggcggcgacgctctcgcccgtgtccagtagggtggcggatggcgcgcggggaccggagcctcctcctcagcgactcggctctgaatcctctgcagtagccgccgaggagcccgac

SEQ ID NO: 16215 - RNA, 587 nt, Homo sapiens
  source 1..587: mol_type = other RNA
gctgggcgaggctggcacagtgtggcaggtcctgggctcaccctacatgaggtacagcagaaatgtctgggccagagtcaaggcttccaatacggacttctcttttccacgtagaggtccagaggtagagagggcaggtttggtgcagaaactgctccatgaagttctcaggaaccgtatctaccagggctcaaccagggaagtagaaccactggtgtctagtggtaggcctctgctggtgataagagatgtcagtgaggaaaaagagctgatcacagagtcgggaagaagagtaagaacgaagtagagaccaggtgcagtggcttatgcctgtaacacagcactttgggaggccgaggtgggaggatcacttgagccgagaagtttgagaacagcatgggcaacaaagtgagacctcgtctctaccaaaataaaaacaaaaaaattagccaggcattttggtgcccgcctgtggccccagctaaacagaagcctgaggcaagaggatcgcttgagcccagaaggtcaagggtgcagtgagccatgttcatgcccctgcaccccagcctgggcaacagagtaaaacc

SEQ ID NO: 16216 - RNA, 245 nt, Homo sapiens
  source 1..245: mol_type = other RNA
gctggtgacatgagaggcccggatgactgcttgttgctgtgtgctgttgtcttttcttagtttctttcctaagttcttccaaaaattctgtctctcagctggtgccctgcagatagagtttcatatccagattcttccactcactattatatgaagagtgggaaaaagagtttaggggagtgggaagagcagtctttggggttatacagagtgcataaattacaactccatgcttcaccacgtat

SEQ ID NO: 16217 - RNA, 404 nt, Homo sapiens
  source 1..404: mol_type = other RNA
ggaggccggggtggggcggggcggcaggagcccgccgtggcgctccgagatgcggggaccgtgcgagcccccaccccattcgctaggcgacggcggcgaccgggaggagcctgcgggcactccggaactggaaggagcttgttgctgtcacgatttgcattttcactgcactgctgtccttaaaaaggaattaccccggtgcccttcagagtcctgtgaaaagtctcagaccgacaggctgccctagatttcactgattatcctaagtccccaaacatgtggttctggggagcattttaaggaattattagcagggcccagggaaaggccctcacataatacattcaaaactaaattttcagagtttttgtttccagattagagcaccaaaaacatgggaaggt

SEQ ID NO: 16218 - RNA, 139 nt, Homo sapiens
  source 1..139: mol_type = other RNA
ggaggccggggtggggcggggcggcgggcacgccgggagctgaggcagtgcctctgggaggacaccacaaccggggcgctttcaggcacactgcggttgcaccacaagcttcctggatggaaggacacgtggccccggg

SEQ ID NO: 16219 - RNA, 1309 nt, Homo sapiens
  source 1..1309: mol_type = other RNA
ggaggccggggtggggcggggcggggcggggctgggctgggaatgttcactggaagaggcactgtcacaagcgtcagagagctgggcatgaggtctgcatggccctgcgggctcttcctacctagaacgcccttccaaggtgaactccacactgcagtcctagacagaggggtgtttctggttggactgtgacatcccagaaagctgtcactcaaaaaaagagtctggggggagggggccggtggtgtaatactacctgttctgctcacttaagccaccagagcagacgccatttcttgcccttcaaagtggggccaaagggtaaatgtgtttggcagacacagctgttcataacatccacctctgggtttgctcgtgtgtttcagaaaacaggtgggtgcaccccttcagttgagggagaaagatttcttcttccttgacaacaatgggttgagtagagttccaattttctccacctcctgcatggccattttccccaagcctgccctcccctaccatacttgatgtctctaagacacactggaacagcggatgcttggggagcccatctgggtgaggaccttgtcaagccactgcaaaggcccattcaggtgcagctcaatccagcagggggtactggtcacagtctgtctcctgtactccgctccccagcctttgacgaagctcatgcggatggtgcacattcgggtcaactggtagacagcctcaaagccctggttgaccgactgggccaggagggcagcgaactcctggttgttgaagatcttcaggttgcatcctggtgggatcttgcagacggtggccgggtgccagccatagcgctggttacagttgggagactggacaaaaatagcgctgtcactgaggcactctgcgaagacctcccctccgatgtagtagagccgcacgcctcttccgatgtgtctccgtgtcagctccactgctgcattcctgttgacattggagagcagccctaggcagaagcgctccgaattggaggggtcggtgaagccatccacagtcatggatggctgcgaggcgtggaatgtctccccgacgcgctggttcagctcgtagtaggagatggagcaccagaaggccggctcgcagtaggtaactggctgcaggtccaagttattatgtgctggggacatcggattcggggataggtttggagaacctgcgtccatgctgtggttcatctggtggtcactggtttctccatcttcactcaggtagccagggggtggggtctccgcgggacgccagggctacccgcaaaggatct

SEQ ID NO: 16220 - RNA, 2045 nt, Homo sapiens
  source 1..2045: mol_type = other RNA
ggaggccggggtggggcggggcggggcggggctgggctgggaatgttcactggaagaggcactgtcacaagcgtcagagagctgggcatgaggtctgcatggccctgcgggctcttcctacctagaacgcccttccaaggtgaactccacactgcagtcctagacagaggggtgtttctggttggactgtgacatcccagaaagctgtcactcaaaaaaagagtctggggggagggggccggtggtgtaatactacctgttctgctcacttaagccaccagagcagacgccatttcttgcccttcaaagtggggccaaagggtaaatgtgtttggcagacacagctgttcataacatccacctctgggtttgctcgtgtgtttcagaaaacaggtgggtgcaccccttcagttgagggagaaagatttcttcttccttgacaacaatgggttgagtagagttccaattttctccacctcctgcatggccattttccccaagcctgccctcccctaccatacttgatgtctctaagacacactggaacagcggatgcttggggagcccatctgggtgaggaccttgtcaagccactgcaaaggcccattcaggtgcagctcaatccagcagggggtactggtcacagtctgtctcctgtactccgctccccagcctttgacgaagctcatgcggatggtgcacattcgggtcaactggtagacagcctcaaagccctggttgaccgactgggccaggagggcagcgaactcctggttgttgaagatcttcaggttgcatcctggtgggatcttgcagacggtggccgggtgccagccatagcgctggttacagttgggagactggacaaaaatagcgctgtcactgaggcactctgcgaagacctcccctccgatgtagtagagccgcacgcctcttccgatgtgtctccgtgtcagctccactgctgcattcctgttgacattggagagcagccctaggcagaagcgctccgaattggaggggtcggtgaagccatccacagtcatggatggctgcgaggcgtggaatgtctccccgacgcgctggttcagctcgtagtaggagatggagcaccagaaggccggctcgcagtaggtaactggctgcaggtccaagttattatgtgctggggacatcggattcggggataggtttggagaacctgcgtccatgctgtggttcatctggtggtcactggtttctccatcttcactcaggtagccagggggtggggtctctggaatattgctctggggctcgatgcctgcggggaagttagtgttttcggggatggaatggctgtagtcgtccagtggggggaactcggccgggatctctgtgtggcgtggcaccaacacaggaggtagaactggtgtctctactctctggtagtggtagggattcacgcagacctcgtccttcttcatattgaaggcgaactcacacagctccatggcccgtagctcgtggtggctgtgcaggtctggccatcgccacaggcggcagtagatgacatgagggagccccttccgatgggacacctgcaaccggccatccagggacagagttgatcctcgctcaggacatacgctctgtccacagtttggggcaaaagtccacatttgtgaagcatttcagaacactgtcccatctccatgggctgcctgaccctcctccacactggccccctcaggaacggagtccaccctcccatccatgtatgccctcccaccgtccccaaatcccccagctgagcaacagtgggccctcagacccccgctggggatgcgtaggaccctccatgcccacttccacctgccttccgggggctgtggaggcctccacaaccaaagcaagcctccccaagtgtcctgtggacagttctctcccaactcccgaagcttgttttctttaattagctcactgtggcaggagaaaaacgcggccccaccctcgaaataagcagatctgggcctcaaatgtactctgtggtttgcctctgtgct

SEQ ID NO: 16221 - RNA, 1682 nt, Homo sapiens
  source 1..1682: mol_type = other RNA
ggaggccggggtggggcggggcggggcggggctgggctgggaatgttcactggaagaggcactgtcacaagcgtcagagagctgggcatgaggtctgcatggccctgcgggctcttcctacctagaacgcccttccaaggtgaactccacactgcagtcctagacagaggggtgtttctggttggactgtgacatcccagaaagctgtcactcaaaaaaagagtctggggggagggggccggtggtgtaatactacctgttctgctcacttaagccaccagagcagacgccatttcttgcccttcaaagtggggccaaagggtaaatgtgtttggcagacacagctgttcataacatccacctctgggtttgctcgtgtgtttcagaaaacaggtgggtgcaccccttcagttgagggagaaagatttcttcttccttgacaacaatgggttgagtagagttccaattttctccacctcctgcatggccattttccccaagcctgccctcccctaccatacttgatgtctctaagacacactggaacagcggatgcttggggagcccatctgggtgaggaccttgtcaagccactgcaaaggcccattcaggtgcagctcaatccagcagggggtactggtcacagtctgtctcctgtactccgctccccagcctttgacgaagctcatgcggatggtgcacattcgggtcaactggtagacagcctcaaagccctggttgaccgactgggccaggagggcagcgaactcctggttgttgaagatcttcaggttgcatcctggtgggatcttgcagacggtggccgggtgccagccatagcgctggttacagttgggagactggacaaaaatagcgctgtcactgaggcactctgcgaagacctcccctccgatgtagtagagccgcacgcctcttccgatgtgtctccgtgtcagctccactgctgcattcctgttgacattggagagcagccctaggcagaagcgctccgaattggaggggtcggtgaagccatccacagtcatggatggctgcgaggcgtggaatgtctccccgacgcgctggttcagctcgtagtaggagatggagcaccagaaggccggctcgcagtaggtaactggctgcaggtccaagttattatgtgctggggacatcggattcggggataggtttggagaacctgcgtccatgctgtggttcatctggtggtcactggtttctccatcttcactcaggtagccagggggtggggtctctggaatattgctctggggctcgatgcctgcggggaagttagtgttttcggggatggaatggctgtagtcgtccagtggggggaactcggccgggatctctgtgtggcgtggcaccaacacaggaggtagaactggtgtctctactctctggtagtggtagggattcacgcagacctcgtccttcttcatattgaaggcgaactcacacagctccatggcccgtagctcgtggtggctgtgcaggtctggccatcgccacaggcggcagtagatgacatgagggagccccttccgatgggacacctgcaaccggccatccagggacctccccatccaccatgctttccggtgtaccagagctgcgcctttccacgtttgcctagggtgcaggcaagacatgtttgt

SEQ ID NO: 16222 - RNA, 2361 nt, Homo sapiens
  source 1..2361: mol_type = other RNA
ggaggccggggtggggcggggcggggcggggctgggctgggaatgttcactggaagaggcactgtcacaagcgtcagagagctgggcatgaggtctgcatggccctgcgggctcttcctacctagaacgcccttccaaggtgaactccacactgcagtcctagacagaggggtgtttctggttggactgtgacatcccagaaagctgtcactcaaaaaaagagtctggggggagggggccggtggtgtaatactacctgttctgctcacttaagccaccagagcagacgccatttcttgcccttcaaagtggggccaaagggtaaatgtgtttggcagacacagctgttcataacatccacctctgggtttgctcgtgtgtttcagaaaacaggtgggtgcaccccttcagttgagggagaaagatttcttcttccttgacaacaatgggttgagtagagttccaattttctccacctcctgcatggccattttccccaagcctgccctcccctaccatacttgatgtctctaagacacactggaacagcggatgcttggggagcccatctgggtgaggaccttgtcaagccactgcaaaggcccattcaggtgcagctcaatccagcagggggtactggtcacagtctgtctcctgtactccgctccccagcctttgacgaagctcatgcggatggtgcacattcgggtcaactggtagacagcctcaaagccctggttgaccgactgggccaggagggcagcgaactcctggttgttgaagatcttcaggttgcatcctggtgggatcttgcagacggtggccgggtgccagccatagcgctggttacagttgggagactggacaaaaatagcgctgtcactgaggcactctgcgaagacctcccctccgatgtagtagagccgcacgcctcttccgatgtgtctccgtgtcagctccactgctgcattcctgttgacattggagagcagccctaggcagaagcgctccgaattggaggggtcggtgaagccatccacagtcatggatggctgcgaggcgtggaatgtctccccgacgcgctggttcagctcgtagtaggagatggagcaccagaaggccggctcgcagtaggtaactggctgcaggtccaagttattatgtgctggggacatcggattcggggataggtttggagaacctgcgtccatgctgtggttcatctggtggtcactggtttctccatcttcactcaggtagccagggggtggggtctctggaatattgctctggggctcgatgcctgcggggaagttagtgttttcggggatggaatggctgtagtcgtccagtggggggaactcggccgggatctctgtgtggcgtggcaccaacacaggaggtagaactggtgtctctactctctggtagtggtagggattcacgcagacctcgtccttcttcatattgaaggcgaactcacacagctccatggcccgtagctcgtggtggctgtgcaggtctggccatcgccacaggcggcagtagatgacatgagggagccccttccgatgggacacctgcaaccggccatccagggacctggggatggtgatgcacttggtgttgacgttctgcgtggtgatggccttctccagctcgtccagctgccccgtcttcttgagtttcttgaccaggctcttgaccgccttctcgcaccatttctcctcctgcccgttctgctcgcccttcttccagcccagcaggcgcttcacgatcgggggagtgaaaggcaggatggacgacatggctggggagggcgcgcgggcggcgaggagcgcccccggcggggctgggctcgacgggacgccgggggcgcagaggggagctcggccggggcctgccgcggtcgcccaaacttcgcctcaactctcggcgaagttgccggggcgccgggccgggccgcggcgctgcagcctgcggggctcggcgcgcggccctgcgcccggagcggctcccacggcgaagagaagagcggccgggcgggcggacggcagcagtgcagggtcgggaaggccccgaacgcggggcggaggcggcggccgcgagactccaagtggcagcagaagtttgggtttccgcacggggtagctgtttgggtgccgcctccgggaaggaaagtccaacccccggccaaacttcgctcgcctcgctagctttgatgcgcagatccctccgcctctgcggcctcaccgccccgccaccctcctcctcccggctcgccgctcgctcgctcgctggctgggccggcccggggcgtgcgccgcgctcccgctcccgcccgctcccagtctgtgtttc

SEQ ID NO: 16223 - RNA, 1845 nt, Homo sapiens
  source 1..1845: mol_type = other RNA
ggaggccggggtggggcggggcggggcggggctgggctgggaatgttcactggaagaggcactgtcacaagcgtcagagagctgggcatgaggtctgcatggccctgcgggctcttcctacctagaacgcccttccaaggtgaactccacactgcagtcctagacagaggggtgtttctggttggactgtgacatcccagaaagctgtcactcaaaaaaagagtctggggggagggggccggtggtgtaatactacctgttctgctcacttaagccaccagagcagacgccatttcttgcccttcaaagtggggccaaagggtaaatgtgtttggcagacacagctgttcataacatccacctctgggtttgctcgtgtgtttcagaaaacaggtgggtgcaccccttcagttgagggagaaagatttcttcttccttgacaacaatgggttgagtagagttccaattttctccacctcctgcatggccattttccccaagcctgccctcccctaccatacttgatgtctctaagacacactggaacagcggatgcttggggagcccatctgggtgaggaccttgtcaagccactgcaaaggcccattcaggtgcagctcaatccagcagggggtactggtcacagtctgtctcctgtactccgctccccagcctttgacgaagctcatgcggatggtgcacattcgggtcaactggtagacagcctcaaagccctggttgaccgactgggccaggagggcagcgaactcctggttgttgaagatcttcaggttgcatcctggtgggatcttgcagacggtggccgggtgccagccatagcgctggttacagttgggagactggacaaaaatagcgctgtcactgaggcactctgcgaagacctcccctccgatgtagtagagccgcacgcctcttccgatgtgtctccgtgtcagctccactgctgcattcctgttgacattggagagcagccctaggcagaagcgctccgaattggaggggtcggtgaagccatccacagtcatggatggctgcgaggcgtggaatgtctccccgacgcgctggttcagctcgtagtaggagatggagcaccagaaggccggctcgcagtaggtaactggctgcaggtccaagttattatgtgctggggacatcggattcggggataggtttggagaacctgcgtccatgctgtggttcatctggtggtcactggtttctccatcttcactcaggtagccagggggtggggtctctggaatattgctctggggctcgatgcctgcggggaagttagtgttttcggggatggaatggctgtagtcgtccagtggggggaactcggccgggatctctgtgtggcgtggcaccaacacaggaggtagaactggtgtctctactctctggtagtggtagggattcacgcagacctcgtccttcttcatattgaaggcgaactcacacagctccatggcccgtagctcgtggtggctgtgcaggtctggccatcgccacaggcggcagtagatgacatgagggagccccttccgatgggacacctgcaaccggccatccagggactcaaacgtggttgctcaacacaggcccgagtgtgggtttccatgcagttgtcccatcctgtgggaatgtcgcatcctgtgggaacccagcgtgtggggttcctggtgaagcgagcggcggcaataaattaccccagtgccgcggctcttgcccacatgttgctcttatggtcagtgcgcttcagcccagcagtgacctaaccccagcaccagtgaactcagcagcaggctcctctgtcatcct

SEQ ID NO: 16224 - RNA, 1718 nt, Homo sapiens
  source 1..1718: mol_type = other RNA
ggaggccggggtggggcggggcggggcggggctgggctgggaatgttcactggaagaggcactgtcacaagcgtcagagagctgggcatgaggtctgcatggccctgcgggctcttcctacctagaacgcccttccaaggtgaactccacactgcagtcctagacagaggggtgtttctggttggactgtgacatcccagaaagctgtcactcaaaaaaagagtctggggggagggggccggtggtgtaatactacctgttctgctcacttaagccaccagagcagacgccatttcttgcccttcaaagtggggccaaagggtaaatgtgtttggcagacacagctgttcataacatccacctctgggtttgctcgtgtgtttcagaaaacaggtgggtgcaccccttcagttgagggagaaagatttcttcttccttgacaacaatgggttgagtagagttccaattttctccacctcctgcatggccattttccccaagcctgccctcccctaccatacttgatgtctctaagacacactggaacagcggatgcttggggagcccatctgggtgaggaccttgtcaagccactgcaaaggcccattcaggtgcagctcaatccagcagggggtactggtcacagtctgtctcctgtactccgctccccagcctttgacgaagctcatgcggatggtgcacattcgggtcaactggtagacagcctcaaagccctggttgaccgactgggccaggagggcagcgaactcctggttgttgaagatcttcaggttgcatcctggtgggatcttgcagacggtggccgggtgccagccatagcgctggttacagttgggagactggacaaaaatagcgctgtcactgaggcactctgcgaagacctcccctccgatgtagtagagccgcacgcctcttccgatgtgtctccgtgtcagctccactgctgcattcctgttgacattggagagcagccctaggcagaagcgctccgaattggaggggtcggtgaagccatccacagtcatggatggctgcgaggcgtggaatgtctccccgacgcgctggttcagctcgtagtaggagatggagcaccagaaggccggctcgcagtaggtaactggctgcaggtccaagttattatgtgctggggacatcggattcggggataggtttggagaacctgcgtccatgctgtggttcatctggtggtcactggtttctccatcttcactcaggtagccagggggtggggtctctggtgtctctactctctggtagtggtagggattcacgcagacctcgtccttcttcatattgaaggcgaactcacacagctccatggcccgtagctcgtggtggctgtgcaggtctggccatcgccacaggcggcagtagatgacatgagggagccccttccgatgggacacctgcaaccggccatccagggacctggggatggtgatgcacttggtgttgacgttctgcgtggtgatggccttctccagctcgtccagctgccccgtcttcttgagtttcttgaccaggctcttgaccgccttctcgcaccatttctcctcctgcccgttctgctcgcccttcttccagcccagcaggcgcttcacgatcgggggagtgaaaggcaggatggacgacatggctggggagggcgcgcgggcggcgaggagcgcccccggcgg

SEQ ID NO: 16225 - RNA, 7238 nt, Homo sapiens
  source 1..7238: mol_type = other RNA
ggaggccggggtggggcggggcgggggcccttcccgggaggagcgaggcagtgggaagtggcacgaaccaagagaaacacgaccccaatgtgggcacccgacgcgcccaaaaccccccaccccgacccccacccccctacacacgagagagacacggcccccctccccactagataacccgaggagacacagtctcccctccccatgggcagacacacccgcccgaaaccccatgggcgggacacagtcccccctcccagagaagtccccagtggagacgccccttaagagactttctcatggccaacacaagccctcccaacacccggagacagccccgacccagggaagaaatggctccagaggccctaccctcgggagagagaggtatcccagggctcctaggagaaaagacaactcagagatgcccagcctcatcctaaagtgctgcagggcagagaaacccccataggagagatgggggtagggccagaaacatcccttcccagacgtgtttcagagatagcccccttccctgggaagagagatggcccgaaactgacttgccttaagtactcccaggaaccctgggaggaaaacaggctccccagagagcctgggtaattgggggagacatgctcccgtggtcctcagcgggaacacatgtcccccggagactcccaaggggagagatagggcctagagagaccccagaggtgagggatgcccagagaacttccccccaccccggaatgtgaaacatgcttcaaggaccctaggagagaaatatgtccccatataccctccccctacggagagacatgccctgaagtagggggatggggaccgactaggtcccctctgggaagacacagactgggtcaggctgggtttgaggggggctctcctctggccaaatgtcgcctattggtacataaaactgtacgcgacacaggcattggggaggggcttcacagacctaggacccacagggatagtccccagtgctgtcgccaacccctgcccacctttggtttcatctctccagtgcccagttggtgacagactcagtgccctggccccaaccagggggctgggggctctgtctttgcctgtgggaagggcttctcagctctcccagccatctgggccaccctctttcttctggcttctccattgtgcaaaatgctcctctgctcttctgctcagtgctcaggggtctctaagaccagggcaaggtacccaggccactaggggcttccagtgggagtccactgaccccaggaatgccgcctgtctggaccaccttctccaccaagcaaatgggcctcatacaatcttcttgcccgaatcctgacctccaggacccaggacaatccttgaggccactgttccaccagctgggcacccaatactaccaactccaagactattgcacctgccccatttgtgcaggggaaaggggctgtctctttaacaagccccaagcccatctcctgggcctccccaagggaaaggagcctttggccaacccctagacctggctgctgccaccccatcccattctaccccttcccctctgtagaagggcttcgtatgccagggctaccagcctaacaatgctctccttcctagcactgtcaccccaagccaagttgggggtaaggggcagataaatagggtgattcttcaggcccctggcttttccggggtgggggtggggtctctggggtacaagagtcaagaccccagcagcacagctcccaaaggcaccagacgaccccgcagcctgtacccaccgctcgcaatcttggaccacctccccaagcttagactaagtcaagcaagggccataccctgagtctccagcctcccagcctgggcccctagggagctggagaggtatgggccaaggcagtgggggtttctggaaggaagaggggctgaggctttgagatggccacagtgggagacgggggctctgcaggacgccccttacaccctggccccctgaggtgaagaagagaacttcacctcatcatggctgactgggcttctctgccccccaacctccctaccccctcccccatgggacccctgaccctgacaaagggaagcccaactggaagaagggggcctggagcccagggtgccctgaggcagccctcccaccccctgagatcaaggcaatggtggttttacaggctgacgggtcagtcatggcaggggctgggggttgagagggcagggagggggcaggatgcaggccccctatatcgggagcagcacccagccaccccctgagcaaaccttcctgctcccaactcacccaaccaggccagaggcacagtcatcccacccctgtccagctgccccccacagcctcagggcccctctgtgatgctcatctggatgtgggaggccagcctgagcggggatccccccagggcacagcgcaacagttccaaaaaaatagagatttgtatttttaagaaaaattaaataaaagcccagctctgctgataggcaaatgttacccccgtccccacccccacccacccgttgtttccctggcctgcacccccatcccaccatggccccaggggtatttacaacatggaacaatagaggcctgggttggggggcactgcggcagggaggagggggcacagggcaggtccccccccagaggggtcccccaagacaacacgacatcaacaagaaaagttgcaaatcaggcagaaatggggacgtcattccaaggtccttatatacagacactgcatgaccagcagggaatgggggcccagatgggactaggcgtgggcatgtggcaggcaggtgggccagtccaggagcagcacgggaaaacaaggcctccgctccactcccacccccgtccctaccccacctttggtaacaaaagcccttcagggagccactggtggtcaagagtttcctctgggagctcccagggaaaggggctccccagttcagccctgcttcagggctaaaattgggcatgctatccccgccctggtcggccatgagggaaacaatgagttagaagtacgctgcccacccttgactccaccatctgcccaaatcgagggggtgctccctggaagtcaagggaaggagcccagtcattgcagaggagccctcttgggcatcagatgggggaagccccataaaggggaaggggcccctgggggctgggagatggaaatgaggggagaggacctggaccctgcatgggagaagggccagcgtggtcatgaggtcagtgatacccccacttggggccctggccaggaagtccacgctgaaggggtggagagtgaggccctggaatgggccatttgggagctggccggcggctgggggaggggggccggccggccagtagggggctcacaggtagatctcgcgcttggccgtctgggcagatgccggtgtggctgcgggtgggaagtccgaggtctgggtcagggggatttcctccaaggtggccgagtccttgcaggaatcatggctactgtgggagaaggcactgtaggagggcaggaggcgcacgggggccgttttggtgttccggtcttccggggggctggggctgccggcgcccgcaggctcctgccctcctcggtcctggtaaggcacgaaggtggagagtttgagggcgctgctcttggtccggcggctgggagatgactggccaggcatccagcatgtgtcagagtggccaaactcactgcactcccgggtacatgtgcctgtcatggcgacatcaggcaaagggcgaaggtcattctcggggtgctccatctctcctatgctgccatcaggggtggtgcgctcatagtgatcctcaggcagggccaggggaccgagtcgaggccctgaggatgacttgctggacggcgtctcagactcctccaggccactgtcatagtaactgtgctgggatgggtcctgcagctcctgggcctggctggtggccgagaaggtgacgcggcggtgaggtaactgcttgctggggtatttgggggggttggtgcggtagctgtagtcggagtactgctcagagcccgtggacgtggtgtccccggtgcccacgaatgtgtttgcaggtggcaggtcctgtaccacctggtgcttcttggaggctgagggtgactggggctgcagctggatggaaggcagtggggagttagagcgatagtggcggcccaggtcagggctgcctggtgggtagttgaggggcaggtggatgcggggactgtccccaggggcatcgctcatcaggttgaacttgagggacttctgcagcccggcctcatcctcgtcctccactggcttcacgggctttggggacttgctcttcttgcctttgcttttgtttcccttggaggccttgccactgggcttgggggcatacaggtccttggtctccttcttaccagcctggtaaccacttttggcctcccgctgtctgcagtagcgcacaagaaccgccagggcgatgagcaaggccacggccaccacaccagccaccacaccaaagagaatgttgccacgctgcttggagcgctcatattctggatccccagcaatgtcaatatccagcggcgtgtccaggctgtggcccaggagggtctccagcagcgtgcggttggccagagtctcattgacataaagatggaccaaggctgtgccatagcgtgggggcttgccgcggtcactgaccttcaccaccaggcggtgtagcccatggtggcgccgctcaatctccttctccagggtgatggcacctgaatgtgacccaatctggaagagtccataagggttgccacctgcaatgctgtagatcagctcagcattgacaccagagtcaaagtcctcggctgccacctggctgaccgtctcaccaagacgtgtctggggggtcagcagcttgtgagaggtgttagaaggggcagtgatatagggtgcgttgtcattctcgtccagcacattgatggtgacaccaacgtaagctgagcgaggtgggacgccaccatccactgccttcagctggaaggtgtaggtgctttgttgctctcgatcaaagctcaggctggataggatggtgcctgtgccattctggataacaaagtcaccgttgtcctgctccactgagagctgcacctgggcattctcccccttgtctccatcaatgacagtcaccatgcccactggactcagtgctggcatgttctccatcactgagaagttgtagccactcagcataaatttggggtcattgtcattgcagtccagcacattgacaaggacagtggctgtgccctggaggctaggactgccccggtcagctgccaccaccttcaactcatagctctcccgctgttcccgatccagagatgtcttcacctggatctctccagtctcgggtgagatggtgaagaggcccttagcagccggctcaggctccagagagtaaaccagctcagcattagagccagagtcagcatcactggcagtgatctcagcaatcacttcaccaggcttgttgttttccgggaaggcgacctcagtgacactctgagtgaagacaggtgcgttgtcattgacgtccaccacctgcaccttgagggagttagtgctggagagtggggggttgccagagtccacagccacaatctcaatggtgtagtctttgaccttctcgtagtctagcggggtggtagtctgcaggaaatacttcttcttgctgtcactgcctgtctcactggcctggcgcagctggaagggcacatcacctgccaccacacaggtgacagctgcattctctccctcatctcggtcagacacctgcaccagggccacagctgtctcctctgccacatcctctgagatgttagccatcccatcttgatgagtcactagccctatgccccggatctcaatggtgggggcattgtcattcatgtccttcacggtcacaaccacctgggcacgggcactcttggggttggtgcctcggtccttagcaagcactgagaagcgcagggtgcttaggtcctcacggtccaccgggccctgaacagtgataagtccagtgttcctgtccagtcgaagaagacgcctcacaacttcgggcgcctggtggaatgtgtattcgatttctgcattggcaccttggtctgagtcattggccttcacctggatgaccgagtggcctatggggctattctcagatagttcggcctcataggagggccgctcaaacttgggggcgttgtcattggtgtcaagcacggtgacacgcagcagggcactgctggcgcgtggggggctgccgccatcctgcaccttgatggtgaggtcataggagtcccagcgctcacggtccaggttgcccatcacaatgagctgtggttgcttctcctcctggtcctctgccacctgcagcccaaatagctcctgggcctcaggcccagcctgcagctcataggatgccacaccgttgggaccagcatcacggtctgaagccagcgggatggggaagagtgagccgatgttggtgttctcagggatggccagagtgatgactggtgaggcgaagttgggtgtgttgtcattgatgtcttgtacttctatctggccctctagcagccgggggctgccattctgcacgaggtctgtgatagatacctcaaactccaggatgcagggatcaccagggagctggttctggcattcacggagcccctcacggtcgatggaggtctcggtggtgaaaatgtcacctgtcttgccatccacgcgaaggtacggggcacccacctctagcttgtacaggtgccccacatctggaaaaccatagtcggctgcgaggctcccaatgagggtgttgggtggctgttcctccggcaccttgtacactacccgagtggcgtggcctggggatggagccagcaggagcagcagtgctagcagcatggagggcagcagtagccgttgccccccagggcctgggctgtgcctcaggtgctccatcctgggaggccccagaatcaggagggcctctcccactgacacacgattctccacaagagcagtcagtcccagcacagaaccccgattccagaaactcagatccctgaatctcatccacagctgggtgtagcagcagtgtctgccccagctggaggagccagtaagaggcctggcat

SEQ ID NO: 16226 - RNA, 6299 nt, Homo sapiens
  source 1..6299: mol_type = other RNA
ggaggccggggtggggcggggcgggggcccttcccgggaggagcgaggcagtgggaagtggcacgaaccaagagaaacacgaccccaatgtgggcacccgacgcgcccaaaaccccccaccccgacccccacccccctacacacgagagagacacggcccccctccccactagataacccgaggagacacagtctcccctccccatgggcagacacacccgcccgaaaccccatgggcgggacacagtcccccctcccagagaagtccccagtggagacgccccttaagagactttctcatggccaacacaagccctcccaacacccggagacagccccgacccagggaagaaatggctccagaggccctaccctcgggagagagaggtatcccagggctcctaggagaaaagacaactcagagatgcccagcctcatcctaaagtgctgcagggcagagaaacccccataggagagatgggggtagggccagaaacatcccttcccagacgtgtttcagagatagcccccttccctgggaagagagatggcccgaaactgacttgccttaagtactcccaggaaccctgggaggaaaacaggctccccagagagcctgggtaattgggggagacatgctcccgtggtcctcagcgggaacacatgtcccccggagactcccaaggggagagatagggcctagagagaccccagaggtgagggatgcccagagaacttccccccaccccggaatgtgaaacatgcttcaaggaccctaggagagaaatatgtccccatataccctccccctacggagagacatgccctgaagtagggggatggggaccgactaggtcccctctgggaagacacagactgggtcaggctgggtttgaggggggctctcctctggccaaatgtcgcctattggtacataaaactgtacgcgacacaggcattggggaggggcttcacagacctaggacccacagggatagtccccagtgctgtcgccaacccctgcccacctttggtttcatctctccagtgcccagttggtgacagactcagtgccctggccccaaccagggggctgggggctctgtctttgcctgtgggaagggcttctcagctctcccagccatctgggccaccctctttcttctggcttctccattgtgcaaaatgctcctctgctcttctgctcagtgctcaggggtctctaagaccagggcaaggtacccaggccactaggggcttccagtgggagtccactgaccccaggaatgccgcctgtctggaccaccttctccaccaagcaaatgggcctcatacaatcttcttgcccgaatcctgacctccaggacccaggacaatccttgaggccactgttccaccagctgggcacccaatactaccaactccaagactattgcacctgccccatttgtgcaggggaaaggggctgtctctttaacaagccccaagcccatctcctgggcctccccaagggaaaggagcctttggccaacccctagacctggctgctgccaccccatcccattctaccccttcccctctgtagaagggcttcgtatgccagggctaccagcctaacaatgctctccttcctagcactgtcaccccaagccaagttgggggtaaggggcagataaatagggtgattcttcaggcccctggcttttccggggtgggggtggggtctctggggtacaagagtcaagaccccagcagcacagctcccaaaggcaccagacgaccccgcagcctgtacccaccgctcgcaatcttggaccacctccccaagcttagactaagtcaagcaagggccataccctgagtctccagcctcccagcctgggcccctagggagctggagaggtatgggccaaggcagtgggggtttctggaaggaagaggggctgaggctttgagatggccacagtgggagacgggggctctgcaggacgccccttacaccctggccccctgaggtgaagaagagaacttcacctcatcatggctgactgggcttctctgccccccaacctccctaccccctcccccatgggacccctgaccctgacaaagggaagcccaactggaagaagggggcctggagcccagggtgccctgaggcagccctcccaccccctgagatcaaggcaatggtggttttacaggctgacgggtcagtcatggcaggggctgggggttgagagggcagggagggggcaggatgcaggccccctatatcgggagcagcacccagccaccccctgagcaaaccttcctgctcccaactcacccaaccaggccagaggcacagtcatcccacccctgtccagctgccccccacagcctcagggcccctctgtgatgctcatctggatgtgggaggccagcctgagcggggatccccccagggcacagcgcaacagttccaaaaaaatagagatttgtatttttaagaaaaattaaataaaagcccagctctgctgataggcaaatgttacccccgtccccacccccacccacccgttgtttccctggcctgcacccccatcccaccatggccccaggggtatttacaacatggaacaatagaggcctgggttggggggcactgcggcagggaggagggggcacagggcaggtccccccccagaggggtcccccaagacaacacgacatcaacaagaaaagttgcaaatcaggcagaaatggggacgtcattccaaggtccttatatacagacactgcatgaccagcagggaatgggggcccagatgggactaggcgtgggcatgtggcaggcaggtgggccagtccaggagcagcacgggaaaacaaggcctccgctccactcccacccccgtccctaccccacctttggtaacaaaagcccttcagggagccactggtggtcaagagtttcctctgggagctcccagggaaaggggctccccagttcagccctgcttcagggctaaaattgggcatgctatccccgccctggtcggccatgagggaaacaatgagttagaagtacgctgcccacccttgactccaccatctgcccaaatcgagggggtgctccctggaagtcaagggaaggagcccagtcattgcagaggagccctcttgggcatcagatgggggaagccccataaaggggaaggggcccctgggggctgggagatggaaatgaggggagaggacctggaccctgcatgggagaagggccagcgtggtcatgaggtcagtgatacccccacttggggccctggccaggaagtccacgctgaaggggtggagagtgaggccctggaatgggccatttgggagctggccggcggctgggggaggggggccggccggccagtagggggctcacaggtagatctcgcgcttggccgtctgggcagatgccggtgtggctgcgggtgggaagtccgaggtctgggtcagggggatttcctccaaggtggccgagtccttgcaggaatcatggctactgtgggagaaggcactgtaggagggcaggaggcgcacgggggccgttttggtgttccggtcttccggggggctggggctgccggcgcccgcaggctcctgccctcctcggtcctggtaaggcacgaaggtggagagtttgagggcgctgctcttggtccggcggctgggagatgactggccaggcatccagcatgtgtcagagtggccaaactcactgcactcccgggtacatgtgcctgtcatggcgacatcaggcaaagggcgaaggtcattctcggggtgctccatctctcctatgctgccatcaggggtggtgcgctcatagtgatcctcaggcagggccaggggaccgagtcgaggccctgaggatgacttgctggacggcgtctcagactcctccaggccactgtcatagtaactgtgctgggatgggtcctgcagctcctgggcctggctggtggccgagaaggtgacgcggcggtgaggtaactgcttgctggggtatttgggggggttggtgcggtagctgtagtcggagtactgctcagagcccgtggacgtggtgtccccggtgcccacgaatgtgtttgcaggtggcaggtcctgtaccacctggtgcttcttggaggctgagggtgactggggctgcagctggatggaaggcagtggggagttagagcgatagtggcggcccaggtcagggctgcctggtgggtagttgaggggcaggtggatgcggggactgtccccaggggcatcgctcatcaggttgaacttgagggacttctgcagcccggcctcatcctcgtcctccactggcttcacgggctttggggacttgctcttcttgcctttgcttttgtttcccttggaggccttgccactgggcttgggggcatacaggtccttggtctccttcttaccagcctggtaaccacttttggcctcccgctgtctgcagtagcgcacaagaaccgccagggcgatgagcaaggccacggccaccacaccagccaccacaccaaagagaatgttgccacgctgcttggagcgctcatattctggatccccagcaatgtcaatatccagcggcgtgtccaggctgtggcccaggagggtctccagcagcgtgcggttggccagagtctcattgacataaagatggaccaaggctgtgccatagcgtgggggcttgccgcggtcactgaccttcaccaccaggcggtgtagcccatggtggcgccgctcaatctccttctccagggtgatggcacctgaatgtgacccaatctggaagagtccataagggttgccacctgcaatgctgtagatcagctcagcattgacaccagagtcaaagtcctcggctgccacctggctgaccgtctcaccaagacgtgtctggggggtcagcagcttgtgagaggtgttagaaggggcagtgatatagggtgcgttgtcattctcgtccagcacattgatggtgacaccaacgtaagctgagcgaggtgggacgccaccatccactgccttcagctggaaggtgtaggtgctttgttgctctcgatcaaagctcaggctggataggatggtgcctgtgccattctggataacaaagtcaccgttgtcctgctccactgagagctgcacctgggcattctcccccttgtctccatcaatgacagtcaccatgcccactggactcagtgctggcatgttctccatcactgagaagttgtagccactcagcataaatttggggtcattgtcattgcagtccagcacattgacaaggacagtggctgtgccctggaggctaggactgccccggtcagctgccaccaccttcaactcatagctctcccgctgttcccgatccagagatgtcttcacctggatctctccagtctcgggtgagatggtgaagaggcccttagcagccggctcaggctccagagagtaaaccagctcagcattagagccagagtcagcatcactggcagtgatctcagcaatcacttcaccaggcttgttgttttccgggaaggcgacctcagtgacactctgagtgaagacaggtgcgttgtcattgacgtccaccacctgcaccttgagggagttagtgctggagagtggggggttgccagagtccacagccacaatctcaatggtgtagtctttgaccttctcgtagtctagcggggtggtagtctgcaggaaatacttcttcttgctgtcactgcctgtctcactggcctggcgcagctggaagggcacatcacctgccaccacacaggtgacagctgcattctctccctcatctcggtcagacacctgcaccagggccacagctgtctcctctgccacatcctctgagatgttagccatcccatcttgatgagtcactagccctatgccccggatctcaatggtgggggcattgtcattcatgtccttcacggtcacaaccacctgggcacgggcactcttggggttggtgcctcggtccttagcaagcactgagaagcgcagggtgcttaggtcctcacggtccaccgggccctgaacagtgataagtccagtgttcctgtccagtcgaagaagacgcctcacaacttcgggcgcctggtggaatgtgtattcgatttctgcattggcaccttggtctgagtcattggccttcacctggttgggtgggctcccatttctagtggtgggtcaccctgacagttatacggagggggcctctcacctggatg

SEQ ID NO: 16227 - RNA, 7233 nt, Homo sapiens
  source 1..7233: mol_type = other RNA
ggaggccggggtggggcggggcgggggcccttcccgggaggagcgaggcagtgggaagtggcacgaaccaagagaaacacgaccccaatgtgggcacccgacgcgcccaaaaccccccaccccgacccccacccccctacacacgagagagacacggcccccctccccactagataacccgaggagacacagtctcccctccccatgggcagacacacccgcccgaaaccccatgggcgggacacagtcccccctcccagagaagtccccagtggagacgccccttaagagactttctcatggccaacacaagccctcccaacacccggagacagccccgacccagggaagaaatggctccagaggccctaccctcgggagagagaggtatcccagggctcctaggagaaaagacaactcagagatgcccagcctcatcctaaagtgctgcagggcagagaaacccccataggagagatgggggtagggccagaaacatcccttcccagacgtgtttcagagatagcccccttccctgggaagagagatggcccgaaactgacttgccttaagtactcccaggaaccctgggaggaaaacaggctccccagagagcctgggtaattgggggagacatgctcccgtggtcctcagcgggaacacatgtcccccggagactcccaaggggagagatagggcctagagagaccccagaggtgagggatgcccagagaacttccccccaccccggaatgtgaaacatgcttcaaggaccctaggagagaaatatgtccccatataccctccccctacggagagacatgccctgaagtagggggatggggaccgactaggtcccctctgggaagacacagactgggtcaggctgggtttgaggggggctctcctctggccaaatgtcgcctattggtacataaaactgtacgcgacacaggcattggggaggggcttcacagacctaggacccacagggatagtccccagtgctgtcgccaacccctgcccacctttggtttcatctctccagtgcccagttggtgacagactcagtgccctggccccaaccagggggctgggggctctgtctttgcctgtgggaagggcttctcagctctcccagccatctgggccaccctctttcttctggcttctccattgtgcaaaatgctcctctgctcttctgctcagtgctcaggggtctctaagaccagggcaaggtacccaggccactaggggcttccagtgggagtccactgaccccaggaatgccgcctgtctggaccaccttctccaccaagcaaatgggcctcatacaatcttcttgcccgaatcctgacctccaggacccaggacaatccttgaggccactgttccaccagctgggcacccaatactaccaactccaagactattgcacctgccccatttgtgcaggggaaaggggctgtctctttaacaagccccaagcccatctcctgggcctccccaagggaaaggagcctttggccaacccctagacctggctgctgccaccccatcccattctaccccttcccctctgtagaagggcttcgtatgccagggctaccagcctaacaatgctctccttcctagcactgtcaccccaagccaagttgggggtaaggggcagataaatagggtgattcttcaggcccctggcttttccggggtgggggtggggtctctggggtacaagagtcaagaccccagcagcacagctcccaaaggcaccagacgaccccgcagcctgtacccaccgctcgcaatcttggaccacctccccaagcttagactaagtcaagcaagggccataccctgagtctccagcctcccagcctgggcccctagggagctggagaggtatgggccaaggcagtgggggtttctggaaggaagaggggctgaggctttgagatggccacagtgggagacgggggctctgcaggacgccccttacaccctggccccctgaggtgaagaagagaacttcacctcatcatggctgactgggcttctctgccccccaacctccctaccccctcccccatgggacccctgaccctgacaaagggaagcccaactggaagaagggggcctggagcccagggtgccctgaggcagccctcccaccccctgagatcaaggcaatggtggttttacaggctgacgggtcagtcatggcaggggctgggggttgagagggcagggagggggcaggatgcaggccccctatatcgggagcagcacccagccaccccctgagcaaaccttcctgctcccaactcacccaaccaggccagaggcacagtcatcccacccctgtccagctgccccccacagcctcagggcccctctgtgatgctcatctggatgtgggaggccagcctgagcggggatccccccagggcacagcgcaacagttccaaaaaaatagagatttgtatttttaagaaaaattaaataaaagcccagctctgctgataggcaaatgttacccccgtccccacccccacccacccgttgtttccctggcctgcacccccatcccaccatggccccaggggtatttacaacatggaacaatagaggcctgggttggggggcactgcggcagggaggagggggcacagggcaggtccccccccagaggggtcccccaagacaacacgacatcaacaagaaaagttgcaaatcaggcagaaatggggacgtcattccaaggtccttatatacagacactgcatgaccagcagggaatgggggcccagatgggactaggcgtgggcatgtggcaggcaggtgggccagtccaggagcagcacgggaaaacaaggcctccgctccactcccacccccgtccctaccccacctttggtaacaaaagcccttcagggagccactggtggtcaagagtttcctctgggagctcccagggaaaggggctccccagttcagccctgcttcagggctaaaattgggcatgctatccccgccctggtcggccatgagggaaacaatgagttagaagtacgctgcccacccttgactccaccatctgcccaaatcgagggggtgctccctggaagtcaagggaaggagcccagtcattgcagaggagccctcttgggcatcagatgggggaagccccataaaggggaaggggcccctgggggctgggagatggaaatgaggggagaggacctggaccctgcatgggagaagggccagcgtggtcatgaggtcagtgatacccccacttggggccctggccaggaagtccacgctgaaggggtggagagtgaggccctggaatgggccatttgggagctggccggcggctgggggaggggggccggccggccagtagggggctcacaggtagatctcgcgcttggccgtctgggcagatgccggtgtggctgcgggtgggaagtccgaggtctgggtcagggggatttcctccaaggtggccgagtccttgcaggaatcatggctactgtgggagaaggcactgtaggagggcaggaggcgcacgggggccgttttggtgttccggtcttccggggggctggggctgccggcgcccgcaggctcctgccctcctcggtcctggtaaggcacgaaggtggagagtttgagggcgctgctcttggtccggcggctgggagatgactggccaggcatccagcatgtgtcagagtggccaaactcactgcactcccgggtacatgtgcctgtcatggcgacatcaggcaaagggcgaaggtcattctcggggtgctccatctctcctatgctgccatcaggggtggtgcgctcatagtgatcctcaggcagggccaggggaccgagtcgaggccctgaggatgacttgctggacggcgtctcagactcctccaggccactgtcatagtaactgtgctgggatgggtcctgcagctcctgggcctggctggtggccgagaaggtgacgcggcggtgaggtaactgcttgctggggtatttgggggggttggtgcggtagctgtagtcggagtactgctcagagcccgtggacgtggtgtccccggtgcccacgaatgtgtttgcaggtggcaggtcctgtaccacctggtgcttcttggaggctgagggtgactggggctgcagctggatggaaggcagtggggagttagagcgatagtggcggcccaggtcagggctgcctggtgggtagttgaggggcaggtggatgcggggactgtccccaggggcatcgctcatcaggttgaacttgagggacttctgcagcccggcctcatcctcgtcctccactggcttcacgggctttggggacttgctcttcttgcctttgcttttgtttcccttggaggccttgccactgggcttgggggcatacaggtccttggtctccttcttaccagcctggtaaccacttttggcctcccgctgtctgcagtagcgcacaagaaccgccagggcgatgagcaaggccacggccaccacaccagccaccacaccaaagagaatgttgccacgctgcttggagcgctcatattctggatccccagcaatgtcaatatccagcggcgtgtccaggctgtggcccaggagggtctccagcagcgtgcggttggccagagtctcattgacataaagatggaccaaggctgtgccatagcgtgggggcttgccgcggtcactgaccttcaccaccaggcggtgtagcccatggtggcgccgctcaatctccttctccagggtgatggcacctgaatgtgacccaatctggaagagtccataagggttgccacctgcaatgctgtagatcagctcagcattgacaccagagtcaaagtcctcggctgccacctggctgaccgtctcaccaagacgtgtctggggggtcagcagcttgtgagaggtgttagaaggggcagtgatatagggtgcgttgtcattctcgtccagcacattgatggtgacaccaacgtaagctgagcgaggtgggacgccaccatccactgccttcagctggaaggtgtaggtgctttgttgctctcgatcaaagctcaggctggataggatggtgcctgtgccattctggataacaaagtcaccgttgtcctgctccactgagagctgcacctgggcattctcccccttgtctccatcaatgacagtcaccatgcccactggactcagtgctggcatgttctccatcactgagaagttgtagccactcagcataaatttggggtcattgtcattgcagtccagcacattgacaaggacagtggctgtgccctggaggctaggactgccccggtcagctgccaccaccttcaactcatagctctcccgctgttcccgatccagagatgtcttcacctggatctctccagtctcgggtgagatggtgaagaggcccttagcagccggctcaggctccagagagtaaaccagctcagcattagagccagagtcagcatcactggcagtgatctcagcaatcacttcaccaggcttgttgttttccgggaaggcgacctcagtgacactctgagtgaagacaggtgcgttgtcattgacgtccaccacctgcaccttgagggagttagtgctggagagtggggggttgccagagtccacagccacaatctcaatggtgtagtctttgaccttctcgtagtctagcggggtggtagtctgcaggaaatacttcttcttgctgtcactgcctgtctcactggcctggcgcagctggaagggcacatcacctgccaccacacaggtgacagctgcattctctccctcatctcggtcagacacctgcaccagggccacagctgtctcctctgccacatcctctgagatgttagccatcccatcttgatgagtcactagccctatgccccggatctcaatggtgggggcattgtcattcatgtccttcacggtcacaaccacctgggcacgggcactcttggggttggtgcctcggtccttagcaagcactgagaagcgcagggtgcttaggtcctcacggtccaccgggccctgaacagtgataagtccagtgttcctgtccagtcgaagaagacgcctcacaacttcgggcgcctggtggaatgtgtattcgatttctgcattggcaccttggtctgagtcattggccttcaccttgtactgtaaggattaaatgatataatacacatcatgtgtttagaacggtgcctggcacctaggctattattatttgctatccccgactgtctgtctcccttttctttctcagtctcttttccaggtcccagtccaccaggctctaaaaaaaaaaaaaaaggctgaaactcccacccatctcccactttggcttgaggacccaggactaagggttttccaggatgggtaatggtgtccagggcaggccgagcctcctcagctccctcacatcaaagagagaggcatcttcagcccatggggaaggggaaaggagctggggctggcaggaggccagagctgagatgacagcgggagatacacccacctgtctgcagagacgctttctttgctccctcccagtccccagccccaccaagctgcctagcgcctggggcagttcccatggagaggggtgctgagaacttcaacagaggaaattgaccccccactgaaccccactgtaccaagcaccccacatctatgggcaccccatgcctaggggaggaggcatgtatacagacaccctagtatgttttttcagaactctgagggtcccacctggctaaaatgatctcatctgactttgtcaggaagaggcaaaatgaggctatatcctccagcttcaggaaaacctcatctggctaaagagaaactatccctggttgggaagatactctcatctcaggagagattctacctggataaacggtgattcctttgttccaactcagctcacctggctagcagagaaggatctacttgactagggcgggagttttacttctcagaggttcccccagcttgagtctgccttaggggtcacgggaaactgttcatatgctatttcactgtcacctaagtagcctgatagaggaaagtaatatcacctgctggggtggggtgggaaagactcccctggctgagtttggggagaaggggtctcactacagtattctggcagttttt

SEQ ID NO: 16228 - RNA, 141 nt, Homo sapiens
  source 1..141: mol_type = other RNA
ggaggccggggtggggcggggcgggggtgggtccctgccctggtggtggtgcctggagacagacagagacaaattcacaagctgaattcctggcaggtcagatggtggggacagttctgcagaaaaaccagccgggagaat

SEQ ID NO: 16229 - RNA, 14258 nt, Homo sapiens
  source 1..14258: mol_type = other RNA
ggaggccggggtggggcggggcgggggtgtgctctctgttccatttgttagttacaggaagctaccaaggatgcacatggtcaagtcactttctacttcccaagttcctccttataacctgagccaaacaatttcaacaatgacaatccattgccccttcagcccagcaggcgactctgacagggaggtgtgaccaccagtctcaaggctgagtggggccttcttgctggctctcgcgctttctgggagtcctgggtgccttggcccagggcagtggtgacagcagggtggaggcagaggtggccccggggacagtgaccctatataaggaagggggcggtgccaggagagattcgtttggagattggttacaaggaagcgagggagagcagaggcagagccctttttcagatacaacatacttacttttcaaatgaacaaaaggcaatttctatgttttaaaaatataagccccaaaaacaatgacacaaaattcatttggttaattcatgtaaaggaaaaaacagcaacaccaccacacaaacaggaaagtgggagtatgattaggaggggtgagatgaaaactattttacagtaacatttccaccaaaagactgtcctaagaacacgctgtcaatacagttcacagggaaaaagcaaatgtggtatttttttgtattttttaaaagctccctggtcccaggtgttttgcagttttcaaggtcttatctgctaaaggaatgccctttaggtcacagcaggtcctctgcagtttggtggtggcacaagagaaaacataaaagaaaccaagactcagggaaactgccattcccccagtctgtttctgcatgacagtggggcccattcctgtctcgaagcatcttcttgttccaaatatgatgtctgtttagagtgggtctcaatggaccaggctgagctgcccctctgtctctgcctcctcctgctcagccctgaccatctctgagaggatgctaaggtccccctcccaccgaactagactttgagtctaagctggacaatgagtaaaacgtaaacatagccttttacattgattttgcttttaaggggaaaacgaataaatgacagcagatatatggaaaacccagccagcgaccatgggaataggggtatatggtcctcccctacaaaacgctgatcaaaatatcacccccggcccagaagtagcagctgtgccttcatggtcacctgaatcccagtctcttctactgcctggtgcctggaaatcagtggatctattaataagttaaatattcaaatcaagacaaaaatcaatgaaccaggttatctgttctcaatgactcttccaagatgtcagagagaaggccttgaagacaagtgtttagacgacacgcatgagaccttcgcatctggcccgggctgcggactcacaccttttccctccatctggattgcctttcatgttctcttgagttcacgtggaaagtaataatccagagggaagtgcgcatgctggactacagaagagtctgggacaacacacttgccttgggggagacacaacctccaactaagaggcattcactggggtttgcggatgtcagttataaacagaacttttctttaaaaagtaccagtctaaatgtaaactataaaacactttaactataaaacgtagccagaaatatgcttaagtatccacagtcaattgtttagtttactcatttaaaatgtgactgttttgatagcttagaaggctaacagcattttacagtagctaaaaacatatatacttaacatgtgcatttgaacatcgcatttgagtacaacacacaaagaataatctcttccttggtttaatttttgttgtaaagatgagctattttcagaattcacttaagcaacgatgaccgggggtatgaagtaatcattattttcagcccacagagaattcatagtctttaaattccaagatcaagctggctacatgatttcaaaaaaggctaaaaccaggatgaatgcccacatttgaggtaattattgccattaggtcacagtttgtgtaagataatgtatctaaaaccttctaaaaaaaaaaaaaatctttaggtgttctgccagaattccagaatacctattgaaaccaaccaggatctcaaactccgattagttaggtttgcttccaatggagttaaagttctaaaagattctagaacttgtgtaaactacctaagaatttaggcaaacaagcctggagccagtcaacaaagaaggttttaaatgaaaaaaggaacaagaaacccactcaaaacaactgaacaaatatttcataataaatgataatagttattttaaaaaattaaaaatctagtcctaagcatttctacattctcaccatctttcaatcaaaataaaaatgcatctgtatttctgttaatctcataccagggcaagagacacgccttccttttatcatgaaagctggctggttttcctgtttatacaattgttgctatttctttgagaagagtatctcaaaagaaaacattcttttgttcctctaagtcttgtctttcttccacctctacttctttttttttttcttttttttttcttttttttaacagaaagaaaaaagttcctggacaccagacccacatatggtatttacaaatttggtgtgaaccctgcctctggttctgcccagagctgaagagtgaatctattacagagatcagagctgtcaggataattatcaagtgcagtaaaaaatagcattttgaaaaaaatatatacctttagtattgcctttctagaattaactataagcaagaaaaacttattttttaaagaagaaaagaatactttttcactcttacttataagagctggttgtagcagcactactaaagctagttggtatgctggaaagaaatctaaaaggaattctatgaatcaaaagaaactctccagagattttctctaaaaatcaaacgaattctgccccttttgcctaaatccaactcaggagccccctctttgcacagtcctttagctgagtcccacggtgcatgggatggcacagggtgatgctgtgtaaaggcctttctttgctcagacatgcaggagacagctgtggctaatggctgcaagctcagttctggagctgggcagactcaggttcaagccctcctcgcccctcaagagttgtgtggctctgggcagtttccttggctgtagggggactaatattgccgatctcacagggctacggagaagatgaaacaggacaacccatgagcaattcccagcacagtgtgtggcatgcaggaagcgggagtatcactaaatggttcatagaaatatgaggccacgcattgctattaattaaaaaaagttaaaagattaaaaatcacatctcaggaagggcctgatgaacaaaaaagggaaccttggggattctggcccatcactgctttatccttccttcaacacctgccacttctcagagcatccggtcagctcccttatctataaatgggggctgttatccccctccctgtgggatggctgttggggccccttgagacaacgctcataaaggccttagcccgggagtcatgaaagcattcaacaaatgttggctattatttacttgagagatattgcaaattttaacaaataagggacagtcagtgtcatgttcaacacagggatctgagatgaggggctcccagaggcttgggcaagtccagcggggggcatcgggaagaccctctctggtgctggtgttctgggacgggagccctgcagggggcacttctctgcaaactctcactgggtttgagggaagaacggcctggagttcttttttgaacttttcagaagctgcaacaagagaaacctctactatgctgggtccctctagtgagccacggtgccaaaagcctccaataggttttttttgcatttaaatcctgtttcaccgccttccattctctagtggcctgagattttactgagtctggtctgtggagatgagaagtgagagttctaaggcatcaaagtggaaaagtactgctattccgagcccagcccccgcgtgctctacgcccttgatgcaactgaactcctggcagccctgctttgctctctcccatggtggcctgggattagtcaagcccacgtattggtatggcaccttgtctcccgatagcagcagcatcgaaggggtcacctccactcctcttaaaagaatagcacagttttgaaataaatgcattttttttttttaaaaaaaaggacagagaggaaagagaaagacaaatagaattgcatcactaatgatgtcattattgcctggaaaggaacgaagggaaggccattttgtccatttctggaggcgtctttgagaagggttctttggctaaagaaaggaacagtttcaccttcctttccaatttggtaaggacatctctggcctgctcaagtttgaagcttccccatcagaagtctgtaaaacacaccagaaggaaaagacacagacagggaatgaagcctgcaaagtccctggggctggaatgtcttgtggccaagtcactcctgctggcgctgtggagtcccaggctggcctgcagaaggaacccttacctctcctcaattctctctgctagttgagagcaccgagccatttccttctttccattttctgtcctagggtctacttgacaggccaacaagagtggtggtcccacaccccaccctgccctcagcatcagacaaagagaacctgggacaaaagctggggcgagctgggtccccacgtcgctctctcaaccatgagccatcagtaatacttcccgaagcctcctcatctcctccctccagtttccaagaaagtttgttccactcactcacacatgctcacacggcctaaatcttccaccccaagcttgttccaatatgagtgtttgccattcccaaggtccaaccaagggaaatcgttctgtcagcagttgggctaatctccccttcccttcctgatgtccatccgtctcacacgttggtgtctgggcgggctgagtcttctaggttgaagaggacaaaggtcagctggctcccccagcccgtgaacacctcagccaccaggaagactagaaaggctaacagtccaggagatgaatgccgctttgctccaacccttctttttcctctgaattccactgaccgcacgctccacttcacagtattaactggcatcaagcctcgactctcccaccccttgatctgctcacccacttcccttggaaacatccaaaacatcatgaagaggccctaagcacagagacatgggggcccacgtccagacgggccagtcagaacccagtgagcagaagcaaattgccctgcggttcaccaggctccagttaaacactcctccgtgacctgacatttcaaatcttcccctcttcctctgaacaatgtctcttcaaatgggaaggagggagcccacaaaagactagaggatgctctagatgattcgtgggctaagtaaggactaggttggcatccctctgcttgagagcttggtcctagtgacagcagcctatttgctaaggtgactcaatggcagattcggccaggtatgcaattgggcatccagggagctggcctctcctgcagggagcttctcttggggcttctgatgtggcagctccatgcatgggggtagaggaggccattgggtgaggactaggagaatgtgcactaatgtttgctgagcgtctgtggggctggcatcgcccaatacttcccttcccttcccttcggtgaagctggctatttcacccctttcttcaactggggcctagcactttgtgggtctggggacagcgtgtgagcacccagcgcacacagcacagtgcactgaagatgtggccggagcccagtggggatgctttcagagggggtgcagcctgtgatgcctgagcagccgcccagctttgttcagggtttctctggcctcctgctgtccctccacccacttccagctggctagaattgggtgctgggggcatgcatcacagggggagggggcaggctgaggaactgggtggtgtggtgaaatttcctggggaaggtaccacctgccagtcactcttacgccacctcactgtgcccagcagcttctgggagggggcaaatgtccctgcattgaagaacctaagccacgccccaggtgcgccgatggcaaaaggatggattgtggggaagcggatggggtcacctctgggagggaattttcttgcttaaataccagaggcaagccaaagatttagttaacagatttcagaagcacaggagagctctgaggatgtgggagagaagctggctaagggctggacagtcagtgactcgacattccccgagcccatgagatgccacctgacgtcgcatcccaggcctctgggatctagaaaatgacaaccttgatggtgaccatgttgtcagaagcccaatcaaggctttgattcttctttaaacttttgttctgtggtggatctttcttgacgtctcttgttgggatagagatgacagaaacaattttcctacttcctaagtctttcctttttttttttgcctgacaaaactggacatctggatgtccctccagtctacttatatactcacagagagaataagtttaaatattaaagagaaaacacaaagatacttggaataaatgtgcatttaaaaccctgactaaaatatcaacataatgatcataattacaatggtaataaaaataattagtacaataatattatctttatgagcagcatggaaatttcattcctgatctggaagaataaaaggaaagaaaatgtcaggtgaaagagtaagtagcctccaacttaagcagacagaataattttctttaaaatgaaaagaacattttaagctgtctttccccctaaaagatcagatctagaaagggctggaaatgaactgtgcccaggaatctgggggtgctctccagtaaggcgaactgaggctcatttgcagccaagacttggaactcgggatgagacctaatgggctattgctgccatctggctgccaaaaagtccctaatagatggattttccaggctgacccagctgtggggcgggggggggtcctctggcttctgtgtcctctgaagcgtttgctgccctcaccctctctgaactgaccattgtcctgctgtctcagagggctgcgcttccccacctccagataaagacagtattgataatggcccgagggaagggaatctccttgctgcaggcctcttgccggcacagcctccagcaggcacttggcaagactgcccggctgtgcccagcatggagcagtcatggtgtccttccttctcgctgaggcctggactaagctgtttccagtttggggacctgtttctttataagtaagaatttatggttggggtggggaagtttccagagttatttcacagctaagagctaagtaacgacttcgttactgagttaggttggatatcactacaaacacacctttcacagtagatccttgagggagactgcacagtgaggaagtaaagggagggaggatgaggatggggccgctgactcgggaaagatctctttgcaccttggaaacctgcctgtggggtcagctaaagactcaacatcagaagcaaacaattagaaccacccttttcggccccatccttggccagattctcctgccattcacattcacatatttcagagttatttactatgaagagagggaactccccacttctccacacctccatccccagaagtgtccaaagcctgagaaaacttccagaatgtatcaaaggtgcaaagagggcaaagggcagatttctttggaaattcaactgtgtgagtttttccaaagtgcagcgtcagacccccggccaccctcataagtgtccctccaaccttctgcccactagaaccctcagaaaccaaaaccaaaatcatgtcttgagcagacctgggtaatgtgaggagagaattcaacagcaaacagaggttggtggttgtctacagagggagggatctggcaagatcgttagagcaaaacagcccagggagccggaggagagagtggagccccgggcgaggctgagagctccaggctctcgtggaggcgggagggactgggggatgccgcctggggcgggagacggctgcctggcgaggccaacagtccggaaacctctggcctcacaaatggcggaactggggacagagtggggcaggggtgaagggtggggagtctctctgggcctccgcccacaaattacaactcaactactgccacaactcaactcccgccgtccccatctccagacgcacccgccgggcatctgtctcccatatttctttcgagatccacggactctctcctagctcctgctggcttccctggcatccttccgctagcaaacagcccaggaaagacaacgggcattaacattttaaaaagaaaaagaaaaagaaaaaaaaaaggccagcgtaaactgttacaacagcacaacagaagagctgagattgtgtctgactagcctcagtttcttggagtaccagtggaagtaaaccctcacgccgcgtctgtcgctcggtaaggcactaggagggaaggatgcagtgtcaagactgcgccagctagggtggcggcgccgagggccacgcggggagggcggcgcgtgcacacccacacgtgctcgctcacccgcacacctgcaccgccacattggttacatgcctatgttatatcgcttttttttgtgcaattacattgaggaatattctattggtatcattggagttgaacacaaggtaggagacaagggtgctgagtgctacattctactagggtgtctgtgacgaccgctagccctacgctacgcgactaggggtggattcaaagagaaaatacattttcagaaaagaaaaaaacctaaagtttgcaacacacattattaatgacatttgagaaacaacgttgcttagggatttatccagagtgctcagaaaaagaaaactcgccccgcgcccccgggggccttccagcagcctggccgtcccccgtctttcctgactagggagcccggactgggcttcgccaatcccacaccagctccaaacatcagcctcctcaggctgcagcccgacattctggagggctgttgaccctttcgagttctggaaaaatccctaaatcttatgttcaattaattaaaaatctatttgatttccatatcaggtgtccctgacagcagtcttccgtatcacttgctgccatatgaaaataatctttgaaaagttcataaagttcttcaaaaactggggccccccgtttctggaatcttcctgttgctctcttctcctttccagtttggcgtagaatgggttcttgagctgggttttttgttattgactttttttttttcctttttcttttttaaaataaaaaccatagatttcccaccctctttaatcccttccttttaaaaatgttctcttctctgctctacgtcctcccacttcccggttcaagtttcactggtgtcccgacccgtccccctgccctctgcccccccccccccccccgcccctgccccgtttgcattgtttgtgtgcggcatcttcagtataaaaggccagcgcccacggtcccaggagcgcctccctccttctctccctcctccctcgggccattctctccctccctccctccctccctcccctccagtgtttatatgtaagggtactggttgaccttggcggggctcagtgggtatccagtgtagacggtggaggctggcgaggcgctgatgtaggtctggtgggcaaattgggctggatactgactcgggtggatggtgggcgagggcaggacccgggggcccatgctcacggggacctggtggacgatgctggctgggtaggcagtgtgctgcacggtgtggcgcgcagagccttgcgaggccaccaggtgggccacggtgccggtggagcccagggccgccggcgcagtgtaggtgtagaggtggggctgggtggggaggtgggcagcggcagcggctgcagccagatgcgggtgcacagtgccgtggctggggctgttgtgcgggaaggagtacggagcctgggccatggtgggagtgatgtaggcctgctgccttcggtggctcccagtgcggtccgtggtgatgtgctgctgagcctggctgagattgagtggctgctgctgctggaagtgggggcccggccgctgctgccggtaggtgatggctccagatgagctccctgaagagtgaccgctggtggaggtcacgttgctggaggacttggacttgtaggaggacgagtggtgactggtgttgactggcaccaggctatcacactccaccaatacttcgctggcctgggttttcaggggtggcacgatgatggttcgggggttccccgtgcagtgattctccaggctccccttggtgtcaaaggcattggcattgttgtgcccagcacgctgctgcacggagtaggggctggtgttgctggaggagtcggagtagggggagtcgtggactgtgacacagctgatgacgttttttctttgcttggagacagtgctggtgggggcgtgtttctgttcctcctcctcgtccgtgtcactgctgatggtgatgacgctgaccgtggggctgggagtgtcgggaatgacaattgtctgccgctgccgttcccgggtggtgctggaggccacgtcgccccacccacaggtgaccgaggtgctgcaggccgggctactgtgcaccatggcacagcggggaggtgtgttctccttgacacgcttggatcgctgtggggagctgatggcctgagaggaggacacctcacaggtggagacatttctcacagatgactggtgctgcttactcttccgggaggaggtggtgctggttggctgctgccgcatcacgtgggccacacccacatttaagggctgtgctgctggaagggtcacatgaccggtcaatagtgcaggctgctgcatgatgggattataatggcttccgtgagcatgcgtatttctccagtccgccagctgctgggtgcctgccatggtctcgggaatcacggtggcatgctgcactgatgtgtgggtggccactccagtcagttgctgccatgctgggggaagcaggatctgctgggtcccacttggccaagcctgctgggcaagcagacctggttggatctgaagaggctgagctcctggggcttgagtgacgatgggaactgcattttccattcgcaccgagtagccagcgtgcttagagggagaggcctgcaagccttggaagccggggggacacacgatgagagcttgctggaacgggtcaggccgggcacaaatctgggctgttcctgtctgcaggggcatgctccgctgggccactgcagccatggatgccgctgagggctggtagagtgtagatgggtagtttagtatggagacttcgggattggctaaggaaatagtggcactggtagaggagggagcctggttgtggacagtggtcagctggttgttaaaggtcatggtcaggttggtggacgtgctgggggccacgtgcgtgatgaaaggggttttgctctggttcaccgtgtcatacatattcacccgacgcttgcagatctccatgttctggaaacatgatttgacgtgtgtgctgtggggaaaatcgagtaagtgtgtcatggtgacaaagggatggttcagggtttcgattggagtgattctcttgtcagcatcaatggtcagcatcttcttcaacaggtcaatgaactcccgccggtcagccttttctaccaacatgtcgctcccttccaaatctgtcgtcatgttcacctgggccatatcatctaaacagttgaaaatgtactttcttgcttcttttgacttaatccctgtctctgcttcatggtcatctggtgtcttcagtctccacaaaggatatggtgagtccgtgtcacggttgaaaaacctagttgtctttgtcccggcgcttaataaatattcagcaggcaaaccctgtgtttgtgaaatataccgaatctgatcatactccgaagctcctggatataacggccaacccaggaacaattctgcaataacacagcccagggaccacatgtcaattgcctcacaaaatggtaaaccaaggatgatctcaggggccctgtaatatctggactgcaagtaggtggagcacacagccttggagacgtggctggctgaaccaaagtcgatgaccttgactctgtatggttgtctagatggatccaccagcatgatgttttctggtttgaggtcagcgtggataagacctaggcttttgagtttcatcagggctgtggctacctgctggagaactgggcgaatgtatttgaggggcaaggggctaaacttgttttgcttcagaaagtcatagaggttctgctccaacatctcgaagaccaagcacgtgtggttcttgtgctggaagcattcgtaggcccggacgaagttatagtcatcggcactctccgtgctcaaccgggccaggatgctcacttcaatctgaccttgtcgggcataggatgggtggttcttcaggatcttgatggctacgatctcattggtgccccgtttccagcacttgaccacttgcccaaacgtccctcggcccaagaactctaagacctcgtaggtgttggtcatggagcacagcacctcatgctgcaccagctgatagtcgccctcgctgttggagccgctgtttttggaggtggcagtagacgtggtggcagtggcgacagtggccccgcttgcattattctgaatcatgggtggatgctcctcgatgatctgcacgctgcttgtgttctcgatctcctcgctcttacgcttgagtccacatttttggtaggtatcaaggaggctcacagtgcttcgacgcattaggttgtgtggtccgccgaggacttgcccggtgacagaagtgctgcttgctgaggtgaccacgatgtgcccggtgcttcctgggaagacgatggtctgctcgtaaggtaggcttgggtttgggaccggcaaggaggtgctgacggttgtggtggctggctgcgacagggggatgttcttgctctggctatacactttgctgtgggagccgtacccagtcatgtcccagttggaactcggctctattttcagtttcttcacactacagaaggcacttgattgaagggtgtgaggggagaaaacttgcacatgtgaggccatacctgggagtggaactgccaggtcaggtggcgactctatgtttaaccttttgaggacctgacacttgttttccaaagtggcctcctgaagtccccaggagtcatgcaaagtcccccagaggtcccaggcaaagcgcacagaaggcccttctgcagagatgctgcccttctgtccttcggtaaaataccagcctaaattcaaagcaggagtcagggtttgtttgatttgaggtaaataaattagagaagctgtgactcgctcagtgccagcagcatgcttagcctggtatcgccccggagaaagagccagcacctggcatggcagacgagggttggcacaatgcatgcttgcttgccagatgaagaggcgctctgtgcaaagtgcagctgcagcaggacgcaaactggtgctctctctaccgtccctcaccagggcaaagctgtctgtgctcctggtcaaagcctcggaggacttatttgctgtcatccacacactgtgctccggaaagtgcctgctcagaaactggcagggagaagacccggagggagtgaggaccatgagaaatcagagagcaactagacaaggaagatatcaaaagagacgggtccttcgaggcctgcacacctgttagtcctaatatatttcagagcaagggatcagactggtgcacacatgggctgaagcccagggaaggagccaagtccaccaccaatgcaactggtgagtcagtatcaggcatgtgtcccctccaagctggcagtaaacaaacactcacacttcatgtttgggcactggactaaattaccaggcaaaagtacaaattccggccaggcgcggtggctcatgcctataatcccagcactttgaga

SEQ ID NO: 16230 - RNA, 13656 nt, Homo sapiens
  source 1..13656: mol_type = other RNA
ggaggccggggtggggcggggcgggggtgtgctctctgttccatttgttagttacaggaagctaccaaggatgcacatggtcaagtcactttctacttcccaagttcctccttataacctgagccaaacaatttcaacaatgacaatccattgccccttcagcccagcaggcgactctgacagggaggtgtgaccaccagtctcaaggctgagtggggccttcttgctggctctcgcgctttctgggagtcctgggtgccttggcccagggcagtggtgacagcagggtggaggcagaggtggccccggggacagtgaccctatataaggaagggggcggtgccaggagagattcgtttggagattggttacaaggaagcgagggagagcagaggcagagccctttttcagatacaacatacttacttttcaaatgaacaaaaggcaatttctatgttttaaaaatataagccccaaaaacaatgacacaaaattcatttggttaattcatgtaaaggaaaaaacagcaacaccaccacacaaacaggaaagtgggagtatgattaggaggggtgagatgaaaactattttacagtaacatttccaccaaaagactgtcctaagaacacgctgtcaatacagttcacagggaaaaagcaaatgtggtatttttttgtattttttaaaagctccctggtcccaggtgttttgcagttttcaaggtcttatctgctaaaggaatgccctttaggtcacagcaggtcctctgcagtttggtggtggcacaagagaaaacataaaagaaaccaagactcagggaaactgccattcccccagtctgtttctgcatgacagtggggcccattcctgtctcgaagcatcttcttgttccaaatatgatgtctgtttagagtgggtctcaatggaccaggctgagctgcccctctgtctctgcctcctcctgctcagccctgaccatctctgagaggatgctaaggtccccctcccaccgaactagactttgagtctaagctggacaatgagtaaaacgtaaacatagccttttacattgattttgcttttaaggggaaaacgaataaatgacagcagatatatggaaaacccagccagcgaccatgggaataggggtatatggtcctcccctacaaaacgctgatcaaaatatcacccccggcccagaagtagcagctgtgccttcatggtcacctgaatcccagtctcttctactgcctggtgcctggaaatcagtggatctattaataagttaaatattcaaatcaagacaaaaatcaatgaaccaggttatctgttctcaatgactcttccaagatgtcagagagaaggccttgaagacaagtgtttagacgacacgcatgagaccttcgcatctggcccgggctgcggactcacaccttttccctccatctggattgcctttcatgttctcttgagttcacgtggaaagtaataatccagagggaagtgcgcatgctggactacagaagagtctgggacaacacacttgccttgggggagacacaacctccaactaagaggcattcactggggtttgcggatgtcagttataaacagaacttttctttaaaaagtaccagtctaaatgtaaactataaaacactttaactataaaacgtagccagaaatatgcttaagtatccacagtcaattgtttagtttactcatttaaaatgtgactgttttgatagcttagaaggctaacagcattttacagtagctaaaaacatatatacttaacatgtgcatttgaacatcgcatttgagtacaacacacaaagaataatctcttccttggtttaatttttgttgtaaagatgagctattttcagaattcacttaagcaacgatgaccgggggtatgaagtaatcattattttcagcccacagagaattcatagtctttaaattccaagatcaagctggctacatgatttcaaaaaaggctaaaaccaggatgaatgcccacatttgaggtaattattgccattaggtcacagtttgtgtaagataatgtatctaaaaccttctaaaaaaaaaaaaaatctttaggtgttctgccagaattccagaatacctattgaaaccaaccaggatctcaaactccgattagttaggtttgcttccaatggagttaaagttctaaaagattctagaacttgtgtaaactacctaagaatttaggcaaacaagcctggagccagtcaacaaagaaggttttaaatgaaaaaaggaacaagaaacccactcaaaacaactgaacaaatatttcataataaatgataatagttattttaaaaaattaaaaatctagtcctaagcatttctacattctcaccatctttcaatcaaaataaaaatgcatctgtatttctgttaatctcataccagggcaagagacacgccttccttttatcatgaaagctggctggttttcctgtttatacaattgttgctatttctttgagaagagtatctcaaaagaaaacattcttttgttcctctaagtcttgtctttcttccacctctacttctttttttttttcttttttttttcttttttttaacagaaagaaaaaagttcctggacaccagacccacatatggtatttacaaatttggtgtgaaccctgcctctggttctgcccagagctgaagagtgaatctattacagagatcagagctgtcaggataattatcaagtgcagtaaaaaatagcattttgaaaaaaatatatacctttagtattgcctttctagaattaactataagcaagaaaaacttattttttaaagaagaaaagaatactttttcactcttacttataagagctggttgtagcagcactactaaagctagttggtatgctggaaagaaatctaaaaggaattctatgaatcaaaagaaactctccagagattttctctaaaaatcaaacgaattctgccccttttgcctaaatccaactcaggagccccctctttgcacagtcctttagctgagtcccacggtgcatgggatggcacagggtgatgctgtgtaaaggcctttctttgctcagacatgcaggagacagctgtggctaatggctgcaagctcagttctggagctgggcagactcaggttcaagccctcctcgcccctcaagagttgtgtggctctgggcagtttccttggctgtagggggactaatattgccgatctcacagggctacggagaagatgaaacaggacaacccatgagcaattcccagcacagtgtgtggcatgcaggaagcgggagtatcactaaatggttcatagaaatatgaggccacgcattgctattaattaaaaaaagttaaaagattaaaaatcacatctcaggaagggcctgatgaacaaaaaagggaaccttggggattctggcccatcactgctttatccttccttcaacacctgccacttctcagagcatccggtcagctcccttatctataaatgggggctgttatccccctccctgtgggatggctgttggggccccttgagacaacgctcataaaggccttagcccgggagtcatgaaagcattcaacaaatgttggctattatttacttgagagatattgcaaattttaacaaataagggacagtcagtgtcatgttcaacacagggatctgagatgaggggctcccagaggcttgggcaagtccagcggggggcatcgggaagaccctctctggtgctggtgttctgggacgggagccctgcagggggcacttctctgcaaactctcactgggtttgagggaagaacggcctggagttcttttttgaacttttcagaagctgcaacaagagaaacctctactatgctgggtccctctagtgagccacggtgccaaaagcctccaataggttttttttgcatttaaatcctgtttcaccgccttccattctctagtggcctgagattttactgagtctggtctgtggagatgagaagtgagagttctaaggcatcaaagtggaaaagtactgctattccgagcccagcccccgcgtgctctacgcccttgatgcaactgaactcctggcagccctgctttgctctctcccatggtggcctgggattagtcaagcccacgtattggtatggcaccttgtctcccgatagcagcagcatcgaaggggtcacctccactcctcttaaaagaatagcacagttttgaaataaatgcattttttttttttaaaaaaaaggacagagaggaaagagaaagacaaatagaattgcatcactaatgatgtcattattgcctggaaaggaacgaagggaaggccattttgtccatttctggaggcgtctttgagaagggttctttggctaaagaaaggaacagtttcaccttcctttccaatttggtaaggacatctctggcctgctcaagtttgaagcttccccatcagaagtctgtaaaacacaccagaaggaaaagacacagacagggaatgaagcctgcaaagtccctggggctggaatgtcttgtggccaagtcactcctgctggcgctgtggagtcccaggctggcctgcagaaggaacccttacctctcctcaattctctctgctagttgagagcaccgagccatttccttctttccattttctgtcctagggtctacttgacaggccaacaagagtggtggtcccacaccccaccctgccctcagcatcagacaaagagaacctgggacaaaagctggggcgagctgggtccccacgtcgctctctcaaccatgagccatcagtaatacttcccgaagcctcctcatctcctccctccagtttccaagaaagtttgttccactcactcacacatgctcacacggcctaaatcttccaccccaagcttgttccaatatgagtgtttgccattcccaaggtccaaccaagggaaatcgttctgtcagcagttgggctaatctccccttcccttcctgatgtccatccgtctcacacgttggtgtctgggcgggctgagtcttctaggttgaagaggacaaaggtcagctggctcccccagcccgtgaacacctcagccaccaggaagactagaaaggctaacagtccaggagatgaatgccgctttgctccaacccttctttttcctctgaattccactgaccgcacgctccacttcacagtattaactggcatcaagcctcgactctcccaccccttgatctgctcacccacttcccttggaaacatccaaaacatcatgaagaggccctaagcacagagacatgggggcccacgtccagacgggccagtcagaacccagtgagcagaagcaaattgccctgcggttcaccaggctccagttaaacactcctccgtgacctgacatttcaaatcttcccctcttcctctgaacaatgtctcttcaaatgggaaggagggagcccacaaaagactagaggatgctctagatgattcgtgggctaagtaaggactaggttggcatccctctgcttgagagcttggtcctagtgacagcagcctatttgctaaggtgactcaatggcagattcggccaggtatgcaattgggcatccagggagctggcctctcctgcagggagcttctcttggggcttctgatgtggcagctccatgcatgggggtagaggaggccattgggtgaggactaggagaatgtgcactaatgtttgctgagcgtctgtggggctggcatcgcccaatacttcccttcccttcccttcggtgaagctggctatttcacccctttcttcaactggggcctagcactttgtgggtctggggacagcgtgtgagcacccagcgcacacagcacagtgcactgaagatgtggccggagcccagtggggatgctttcagagggggtgcagcctgtgatgcctgagcagccgcccagctttgttcagggtttctctggcctcctgctgtccctccacccacttccagctggctagaattgggtgctgggggcatgcatcacagggggagggggcaggctgaggaactgggtggtgtggtgaaatttcctggggaaggtaccacctgccagtcactcttacgccacctcactgtgcccagcagcttctgggagggggcaaatgtccctgcattgaagaacctaagccacgccccaggtgcgccgatggcaaaaggatggattgtggggaagcggatggggtcacctctgggagggaattttcttgcttaaataccagaggcaagccaaagatttagttaacagatttcagaagcacaggagagctctgaggatgtgggagagaagctggctaagggctggacagtcagtgactcgacattccccgagcccatgagatgccacctgacgtcgcatcccaggcctctgggatctagaaaatgacaaccttgatggtgaccatgttgtcagaagcccaatcaaggctttgattcttctttaaacttttgttctgtggtggatctttcttgacgtctcttgttgggatagagatgacagaaacaattttcctacttcctaagtctttcctttttttttttgcctgacaaaactggacatctggatgtccctccagtctacttatatactcacagagagaataagtttaaatattaaagagaaaacacaaagatacttggaataaatgtgcatttaaaaccctgactaaaatatcaacataatgatcataattacaatggtaataaaaataattagtacaataatattatctttatgagcagcatggaaatttcattcctgatctggaagaataaaaggaaagaaaatgtcaggtgaaagagtaagtagcctccaacttaagcagacagaataattttctttaaaatgaaaagaacattttaagctgtctttccccctaaaagatcagatctagaaagggctggaaatgaactgtgcccaggaatctgggggtgctctccagtaaggcgaactgaggctcatttgcagccaagacttggaactcgggatgagacctaatgggctattgctgccatctggctgccaaaaagtccctaatagatggattttccaggctgacccagctgtggggcgggggggggtcctctggcttctgtgtcctctgaagcgtttgctgccctcaccctctctgaactgaccattgtcctgctgtctcagagggctgcgcttccccacctccagataaagacagtattgataatggcccgagggaagggaatctccttgctgcaggcctcttgccggcacagcctccagcaggcacttggcaagactgcccggctgtgcccagcatggagcagtcatggtgtccttccttctcgctgaggcctggactaagctgtttccagtttggggacctgtttctttataagtaagaatttatggttggggtggggaagtttccagagttatttcacagctaagagctaagtaacgacttcgttactgagttaggttggatatcactacaaacacacctttcacagtagatccttgagggagactgcacagtgaggaagtaaagggagggaggatgaggatggggccgctgactcgggaaagatctctttgcaccttggaaacctgcctgtggggtcagctaaagactcaacatcagaagcaaacaattagaaccacccttttcggccccatccttggccagattctcctgccattcacattcacatatttcagagttatttactatgaagagagggaactccccacttctccacacctccatccccagaagtgtccaaagcctgagaaaacttccagaatgtatcaaaggtgcaaagagggcaaagggcagatttctttggaaattcaactgtgtgagtttttccaaagtgcagcgtcagacccccggccaccctcataagtgtccctccaaccttctgcccactagaaccctcagaaaccaaaaccaaaatcatgtcttgagcagacctgggtaatgtgaggagagaattcaacagcaaacagaggttggtggttgtctacagagggagggatctggcaagatcgttagagcaaaacagcccagggagccggaggagagagtggagccccgggcgaggctgagagctccaggctctcgtggaggcgggagggactgggggatgccgcctggggcgggagacggctgcctggcgaggccaacagtccggaaacctctggcctcacaaatggcggaactggggacagagtggggcaggggtgaagggtggggagtctctctgggcctccgcccacaaattacaactcaactactgccacaactcaactcccgccgtccccatctccagacgcacccgccgggcatctgtctcccatatttctttcgagatccacggactctctcctagctcctgctggcttccctggcatccttccgctagcaaacagcccaggaaagacaacgggcattaacattttaaaaagaaaaagaaaaagaaaaaaaaaaggccagcgtaaactgttacaacagcacaacagaagagctgagattgtgtctgactagcctcagtttcttggagtaccagtggaagtaaaccctcacgccgcgtctgtcgctcggtaaggcactaggagggaaggatgcagtgtcaagactgcgccagctagggtggcggcgccgagggccacgcggggagggcggcgcgtgcacacccacacgtgctcgctcacccgcacacctgcaccgccacattggttacatgcctatgttatatcgcttttttttgtgcaattacattgaggaatattctattggtatcattggagttgaacacaaggtaggagacaagggtgctgagtgctacattctactagggtgtctgtgacgaccgctagccctacgctacgcgactaggggtggattcaaagagaaaatacattttcagaaaagaaaaaaacctaaagtttgcaacacacattattaatgacatttgagaaacaacgttgcttagggatttatccagagtgctcagaaaaagaaaactcgccccgcgcccccgggggccttccagcagcctggccgtcccccgtctttcctgactagggagcccggactgggcttcgccaatcccacaccagctccaaacatcagcctcctcaggctgcagcccgacattctggagggctgttgaccctttcgagttctggaaaaatccctaaatcttatgttcaattaattaaaaatctatttgatttccatatcaggtgtccctgacagcagtcttccgtatcacttgctgccatatgaaaataatctttgaaaagttcataaagttcttcaaaaactggggccccccgtttctggaatcttcctgttgctctcttctcctttccagtttggcgtagaatgggttcttgagctgggttttttgttattgactttttttttttcctttttcttttttaaaataaaaaccatagatttcccaccctctttaatcccttccttttaaaaatgttctcttctctgctctacgtcctcccacttcccggttcaagtttcactggtgtcccgacccgtccccctgccctctgcccccccccccccccccgcccctgccccgtttgcattgtttgtgtgcggcatcttcagtataaaaggccagcgcccacggtcccaggagcgcctccctccttctctccctcctccctcgggccattctctccctccctccctccctccctcccctccagtgtttatatgtaagggtactggttgaccttggcggggctcagtgggtatccagtgtagacggtggaggctggcgaggcgctgatgtaggtctggtgggcaaattgggctggatactgactcgggtggatggtgggcgagggcaggacccgggggcccatgctcacggggacctggtggacgatgctggctgggtaggcagtgtgctgcacggtgtggcgcgcagagccttgcgaggccaccaggtgggccacggtgccggtggagcccagggccgccggcgcagtgtaggtgtagaggtggggctgggtggggaggtgggcagcggcagcggctgcagccagatgcgggtgcacagtgccgtggctggggctgttgtgcgggaaggagtacggagcctgggccatggtgggagtgatgtaggcctgctgccttcggtggctcccagtgcggtccgtggtgatgtgctgctgagcctggctgagattgagtggctgctgctgctggaagtgggggcccggccgctgctgccggtaggtgatggctccagatgagctccctgaagagtgaccgctggtggaggtcacgttgctggaggacttggacttgtaggaggacgagtggtgactggtgttgactggcaccaggctatcacactccaccaatacttcgctggcctgggttttcaggggtggcacgatgatggttcgggggttccccgtgcagtgattctccaggctccccttggtgtcaaaggcattggcattgttgtgcccagcacgctgctgcacggagtaggggctggtgttgctggaggagtcggagtagggggagtcgtggactgtgacacagctgatgacgttttttctttgcttggagacagtgctggtgggggcgtgtttctgttcctcctcctcgtccgtgtcactgctgatggtgatgacgctgaccgtggggctgggagtgtcgggaatgacaattgtctgccgctgccgttcccgggtggtgctggaggccacgtcgccccacccacaggtgaccgaggtgctgcaggccgggctactgtgcaccatggcacagcggggaggtgtgttctccttgacacgcttggatcgctgtggggagctgatggcctgagaggaggacacctcacaggtggagacatttctcacagatgactggtgctgcttactcttccgggaggaggtggtgctggttggctgctgccgcatcacgtgggccacacccacatttaagggctgtgctgctggaagggtcacatgaccggtcaatagtgcaggctgctgcatgatgggattataatggcttccgtgagcatgcgtatttctccagtccgccagctgctgggtgcctgccatggtctcgggaatcacggtggcatgctgcactgatgtgtgggtggccactccagtcagttgctgccatgctgggggaagcaggatctgctgggtcccacttggccaagcctgctgggcaagcagacctggttggatctgaagaggctgagctcctggggcttgagtgacgatgggaactgcattttccattcgcaccgagtagccagcgtgcttagagggagaggcctgcaagccttggaagccggggggacacacgatgagagcttgctggaacgggtcaggccgggcacaaatctgggctgttcctgtctgcaggggcatgctccgctgggccactgcagccatggatgccgctgagggctggtagagtgtagatgggtagtttagtatggagacttcgggattggctaaggaaatagtggcactggtagaggagggagcctggttgtggacagtggtcagctggttgttaaaggtcatggtcaggttggtggacgtgctgggggccacgtgcgtgatgaaaggggttttgctctggttcaccgtgtcatacatattcacccgacgcttgcagatctccatgttctggaaacatgatttgacgtgtgtgctgtggggaaaatcgagtaagtgtgtcatggtgacaaagggatggttcagggtttcgattggagtgattctcttgtcagcatcaatggtcagcatcttcttcaacaggtcaatgaactcccgccggtcagccttttctaccaacatgtcgctcccttccaaatctgtcgtcatgttcacctgggccatatcatctaaacagttgaaaatgtactttcttgcttcttttgacttaatccctgtctctgcttcatggtcatctggtgtcttcagtctccacaaaggatatggtgagtccgtgtcacggttgaaaaacctagttgtctttgtcccggcgcttaataaatattcagcaggcaaaccctgtgtttgtgaaatataccgaatctgatcatactccgaagctcctggatataacggccaacccaggaacaattctgcaataacacagcccagggaccacatgtcaattgcctcacaaaatggtaaaccaaggatgatctcaggggccctgtaatatctggactgcaagtaggtggagcacacagccttggagacgtggctggctgaaccaaagtcgatgaccttgactctgtatggttgtctagatggatccaccagcatgatgttttctggtttgaggtcagcgtggataagacctaggcttttgagtttcatcagggctgtggctacctgctggagaactgggcgaatgtatttgaggggcaaggggctaaacttgttttgcttcagaaagtcatagaggttctgctccaacatctcgaagaccaagcacgtgtggttcttgtgctggaagcattcgtaggcccggacgaagttatagtcatcggcactctccgtgctcaaccgggccaggatgctcacttcaatctgaccttgtcgggcataggatgggtggttcttcaggatcttgatggctacgatctcattggtgccccgtttccagcacttgaccacttgcccaaacgtccctcggcccaagaactctaagacctcgtaggtgttggtcatggagcacagcacctcatgctgcaccagctgatagtcgccctcgctgttggagccgctgtttttggaggtggcagtagacgtggtggcagtggcgacagtggccccgcttgcattattctgaatcatgggtggatgctcctcgatgatctgcacgctgcttgtgttctcgatctcctcgctcttacgcttgagtccacatttttggtaggtatcaaggaggctcacagtgcttcgacgcattaggttgtgtggtccgccgaggacttgcccggtgacagaagtgctgcttgctgaggtgaccacgatgtgcccggtgcttcctgggaagacgatggtctgctcgtaaggtaggcttgggtttgggaccggcaaggaggtgctgacggttgtggtggctggctgcgacagggggatgttcttgctctggctatacactttgctgtgggagccgtacccagtcatgtcccagttggaactcggctctattttcagtttcttcacactacagaaggcacttgattgaagggtgtgaggggagaaaacttgcacatgtgaggccatacctgtgatcaatggtttatgctcccttttcttcaatgcccacatcttaatccatctcccccaactcgttaatgcactataggctcctgttcttgaaggtaaatgacttcctaattgcctaatccaatggccttgtttcagcccgttcttcttaacctctgcaacatctgatactgctgaccacgacttccttcttgatgctcttctctggacttcagtgaatctgtaatctccccatcccgtgtctgattgcacactgtgtgctcg

SEQ ID NO: 16231 - RNA, 13785 nt, Homo sapiens
  source 1..13785: mol_type = other RNA
ggaggccggggtggggcggggcgggggtgtgctctctgttccatttgttagttacaggaagctaccaaggatgcacatggtcaagtcactttctacttcccaagttcctccttataacctgagccaaacaatttcaacaatgacaatccattgccccttcagcccagcaggcgactctgacagggaggtgtgaccaccagtctcaaggctgagtggggccttcttgctggctctcgcgctttctgggagtcctgggtgccttggcccagggcagtggtgacagcagggtggaggcagaggtggccccggggacagtgaccctatataaggaagggggcggtgccaggagagattcgtttggagattggttacaaggaagcgagggagagcagaggcagagccctttttcagatacaacatacttacttttcaaatgaacaaaaggcaatttctatgttttaaaaatataagccccaaaaacaatgacacaaaattcatttggttaattcatgtaaaggaaaaaacagcaacaccaccacacaaacaggaaagtgggagtatgattaggaggggtgagatgaaaactattttacagtaacatttccaccaaaagactgtcctaagaacacgctgtcaatacagttcacagggaaaaagcaaatgtggtatttttttgtattttttaaaagctccctggtcccaggtgttttgcagttttcaaggtcttatctgctaaaggaatgccctttaggtcacagcaggtcctctgcagtttggtggtggcacaagagaaaacataaaagaaaccaagactcagggaaactgccattcccccagtctgtttctgcatgacagtggggcccattcctgtctcgaagcatcttcttgttccaaatatgatgtctgtttagagtgggtctcaatggaccaggctgagctgcccctctgtctctgcctcctcctgctcagccctgaccatctctgagaggatgctaaggtccccctcccaccgaactagactttgagtctaagctggacaatgagtaaaacgtaaacatagccttttacattgattttgcttttaaggggaaaacgaataaatgacagcagatatatggaaaacccagccagcgaccatgggaataggggtatatggtcctcccctacaaaacgctgatcaaaatatcacccccggcccagaagtagcagctgtgccttcatggtcacctgaatcccagtctcttctactgcctggtgcctggaaatcagtggatctattaataagttaaatattcaaatcaagacaaaaatcaatgaaccaggttatctgttctcaatgactcttccaagatgtcagagagaaggccttgaagacaagtgtttagacgacacgcatgagaccttcgcatctggcccgggctgcggactcacaccttttccctccatctggattgcctttcatgttctcttgagttcacgtggaaagtaataatccagagggaagtgcgcatgctggactacagaagagtctgggacaacacacttgccttgggggagacacaacctccaactaagaggcattcactggggtttgcggatgtcagttataaacagaacttttctttaaaaagtaccagtctaaatgtaaactataaaacactttaactataaaacgtagccagaaatatgcttaagtatccacagtcaattgtttagtttactcatttaaaatgtgactgttttgatagcttagaaggctaacagcattttacagtagctaaaaacatatatacttaacatgtgcatttgaacatcgcatttgagtacaacacacaaagaataatctcttccttggtttaatttttgttgtaaagatgagctattttcagaattcacttaagcaacgatgaccgggggtatgaagtaatcattattttcagcccacagagaattcatagtctttaaattccaagatcaagctggctacatgatttcaaaaaaggctaaaaccaggatgaatgcccacatttgaggtaattattgccattaggtcacagtttgtgtaagataatgtatctaaaaccttctaaaaaaaaaaaaaatctttaggtgttctgccagaattccagaatacctattgaaaccaaccaggatctcaaactccgattagttaggtttgcttccaatggagttaaagttctaaaagattctagaacttgtgtaaactacctaagaatttaggcaaacaagcctggagccagtcaacaaagaaggttttaaatgaaaaaaggaacaagaaacccactcaaaacaactgaacaaatatttcataataaatgataatagttattttaaaaaattaaaaatctagtcctaagcatttctacattctcaccatctttcaatcaaaataaaaatgcatctgtatttctgttaatctcataccagggcaagagacacgccttccttttatcatgaaagctggctggttttcctgtttatacaattgttgctatttctttgagaagagtatctcaaaagaaaacattcttttgttcctctaagtcttgtctttcttccacctctacttctttttttttttcttttttttttcttttttttaacagaaagaaaaaagttcctggacaccagacccacatatggtatttacaaatttggtgtgaaccctgcctctggttctgcccagagctgaagagtgaatctattacagagatcagagctgtcaggataattatcaagtgcagtaaaaaatagcattttgaaaaaaatatatacctttagtattgcctttctagaattaactataagcaagaaaaacttattttttaaagaagaaaagaatactttttcactcttacttataagagctggttgtagcagcactactaaagctagttggtatgctggaaagaaatctaaaaggaattctatgaatcaaaagaaactctccagagattttctctaaaaatcaaacgaattctgccccttttgcctaaatccaactcaggagccccctctttgcacagtcctttagctgagtcccacggtgcatgggatggcacagggtgatgctgtgtaaaggcctttctttgctcagacatgcaggagacagctgtggctaatggctgcaagctcagttctggagctgggcagactcaggttcaagccctcctcgcccctcaagagttgtgtggctctgggcagtttccttggctgtagggggactaatattgccgatctcacagggctacggagaagatgaaacaggacaacccatgagcaattcccagcacagtgtgtggcatgcaggaagcgggagtatcactaaatggttcatagaaatatgaggccacgcattgctattaattaaaaaaagttaaaagattaaaaatcacatctcaggaagggcctgatgaacaaaaaagggaaccttggggattctggcccatcactgctttatccttccttcaacacctgccacttctcagagcatccggtcagctcccttatctataaatgggggctgttatccccctccctgtgggatggctgttggggccccttgagacaacgctcataaaggccttagcccgggagtcatgaaagcattcaacaaatgttggctattatttacttgagagatattgcaaattttaacaaataagggacagtcagtgtcatgttcaacacagggatctgagatgaggggctcccagaggcttgggcaagtccagcggggggcatcgggaagaccctctctggtgctggtgttctgggacgggagccctgcagggggcacttctctgcaaactctcactgggtttgagggaagaacggcctggagttcttttttgaacttttcagaagctgcaacaagagaaacctctactatgctgggtccctctagtgagccacggtgccaaaagcctccaataggttttttttgcatttaaatcctgtttcaccgccttccattctctagtggcctgagattttactgagtctggtctgtggagatgagaagtgagagttctaaggcatcaaagtggaaaagtactgctattccgagcccagcccccgcgtgctctacgcccttgatgcaactgaactcctggcagccctgctttgctctctcccatggtggcctgggattagtcaagcccacgtattggtatggcaccttgtctcccgatagcagcagcatcgaaggggtcacctccactcctcttaaaagaatagcacagttttgaaataaatgcattttttttttttaaaaaaaaggacagagaggaaagagaaagacaaatagaattgcatcactaatgatgtcattattgcctggaaaggaacgaagggaaggccattttgtccatttctggaggcgtctttgagaagggttctttggctaaagaaaggaacagtttcaccttcctttccaatttggtaaggacatctctggcctgctcaagtttgaagcttccccatcagaagtctgtaaaacacaccagaaggaaaagacacagacagggaatgaagcctgcaaagtccctggggctggaatgtcttgtggccaagtcactcctgctggcgctgtggagtcccaggctggcctgcagaaggaacccttacctctcctcaattctctctgctagttgagagcaccgagccatttccttctttccattttctgtcctagggtctacttgacaggccaacaagagtggtggtcccacaccccaccctgccctcagcatcagacaaagagaacctgggacaaaagctggggcgagctgggtccccacgtcgctctctcaaccatgagccatcagtaatacttcccgaagcctcctcatctcctccctccagtttccaagaaagtttgttccactcactcacacatgctcacacggcctaaatcttccaccccaagcttgttccaatatgagtgtttgccattcccaaggtccaaccaagggaaatcgttctgtcagcagttgggctaatctccccttcccttcctgatgtccatccgtctcacacgttggtgtctgggcgggctgagtcttctaggttgaagaggacaaaggtcagctggctcccccagcccgtgaacacctcagccaccaggaagactagaaaggctaacagtccaggagatgaatgccgctttgctccaacccttctttttcctctgaattccactgaccgcacgctccacttcacagtattaactggcatcaagcctcgactctcccaccccttgatctgctcacccacttcccttggaaacatccaaaacatcatgaagaggccctaagcacagagacatgggggcccacgtccagacgggccagtcagaacccagtgagcagaagcaaattgccctgcggttcaccaggctccagttaaacactcctccgtgacctgacatttcaaatcttcccctcttcctctgaacaatgtctcttcaaatgggaaggagggagcccacaaaagactagaggatgctctagatgattcgtgggctaagtaaggactaggttggcatccctctgcttgagagcttggtcctagtgacagcagcctatttgctaaggtgactcaatggcagattcggccaggtatgcaattgggcatccagggagctggcctctcctgcagggagcttctcttggggcttctgatgtggcagctccatgcatgggggtagaggaggccattgggtgaggactaggagaatgtgcactaatgtttgctgagcgtctgtggggctggcatcgcccaatacttcccttcccttcccttcggtgaagctggctatttcacccctttcttcaactggggcctagcactttgtgggtctggggacagcgtgtgagcacccagcgcacacagcacagtgcactgaagatgtggccggagcccagtggggatgctttcagagggggtgcagcctgtgatgcctgagcagccgcccagctttgttcagggtttctctggcctcctgctgtccctccacccacttccagctggctagaattgggtgctgggggcatgcatcacagggggagggggcaggctgaggaactgggtggtgtggtgaaatttcctggggaaggtaccacctgccagtcactcttacgccacctcactgtgcccagcagcttctgggagggggcaaatgtccctgcattgaagaacctaagccacgccccaggtgcgccgatggcaaaaggatggattgtggggaagcggatggggtcacctctgggagggaattttcttgcttaaataccagaggcaagccaaagatttagttaacagatttcagaagcacaggagagctctgaggatgtgggagagaagctggctaagggctggacagtcagtgactcgacattccccgagcccatgagatgccacctgacgtcgcatcccaggcctctgggatctagaaaatgacaaccttgatggtgaccatgttgtcagaagcccaatcaaggctttgattcttctttaaacttttgttctgtggtggatctttcttgacgtctcttgttgggatagagatgacagaaacaattttcctacttcctaagtctttcctttttttttttgcctgacaaaactggacatctggatgtccctccagtctacttatatactcacagagagaataagtttaaatattaaagagaaaacacaaagatacttggaataaatgtgcatttaaaaccctgactaaaatatcaacataatgatcataattacaatggtaataaaaataattagtacaataatattatctttatgagcagcatggaaatttcattcctgatctggaagaataaaaggaaagaaaatgtcaggtgaaagagtaagtagcctccaacttaagcagacagaataattttctttaaaatgaaaagaacattttaagctgtctttccccctaaaagatcagatctagaaagggctggaaatgaactgtgcccaggaatctgggggtgctctccagtaaggcgaactgaggctcatttgcagccaagacttggaactcgggatgagacctaatgggctattgctgccatctggctgccaaaaagtccctaatagatggattttccaggctgacccagctgtggggcgggggggggtcctctggcttctgtgtcctctgaagcgtttgctgccctcaccctctctgaactgaccattgtcctgctgtctcagagggctgcgcttccccacctccagataaagacagtattgataatggcccgagggaagggaatctccttgctgcaggcctcttgccggcacagcctccagcaggcacttggcaagactgcccggctgtgcccagcatggagcagtcatggtgtccttccttctcgctgaggcctggactaagctgtttccagtttggggacctgtttctttataagtaagaatttatggttggggtggggaagtttccagagttatttcacagctaagagctaagtaacgacttcgttactgagttaggttggatatcactacaaacacacctttcacagtagatccttgagggagactgcacagtgaggaagtaaagggagggaggatgaggatggggccgctgactcgggaaagatctctttgcaccttggaaacctgcctgtggggtcagctaaagactcaacatcagaagcaaacaattagaaccacccttttcggccccatccttggccagattctcctgccattcacattcacatatttcagagttatttactatgaagagagggaactccccacttctccacacctccatccccagaagtgtccaaagcctgagaaaacttccagaatgtatcaaaggtgcaaagagggcaaagggcagatttctttggaaattcaactgtgtgagtttttccaaagtgcagcgtcagacccccggccaccctcataagtgtccctccaaccttctgcccactagaaccctcagaaaccaaaaccaaaatcatgtcttgagcagacctgggtaatgtgaggagagaattcaacagcaaacagaggttggtggttgtctacagagggagggatctggcaagatcgttagagcaaaacagcccagggagccggaggagagagtggagccccgggcgaggctgagagctccaggctctcgtggaggcgggagggactgggggatgccgcctggggcgggagacggctgcctggcgaggccaacagtccggaaacctctggcctcacaaatggcggaactggggacagagtggggcaggggtgaagggtggggagtctctctgggcctccgcccacaaattacaactcaactactgccacaactcaactcccgccgtccccatctccagacgcacccgccgggcatctgtctcccatatttctttcgagatccacggactctctcctagctcctgctggcttccctggcatccttccgctagcaaacagcccaggaaagacaacgggcattaacattttaaaaagaaaaagaaaaagaaaaaaaaaaggccagcgtaaactgttacaacagcacaacagaagagctgagattgtgtctgactagcctcagtttcttggagtaccagtggaagtaaaccctcacgccgcgtctgtcgctcggtaaggcactaggagggaaggatgcagtgtcaagactgcgccagctagggtggcggcgccgagggccacgcggggagggcggcgcgtgcacacccacacgtgctcgctcacccgcacacctgcaccgccacattggttacatgcctatgttatatcgcttttttttgtgcaattacattgaggaatattctattggtatcattggagttgaacacaaggtaggagacaagggtgctgagtgctacattctactagggtgtctgtgacgaccgctagccctacgctacgcgactaggggtggattcaaagagaaaatacattttcagaaaagaaaaaaacctaaagtttgcaacacacattattaatgacatttgagaaacaacgttgcttagggatttatccagagtgctcagaaaaagaaaactcgccccgcgcccccgggggccttccagcagcctggccgtcccccgtctttcctgactagggagcccggactgggcttcgccaatcccacaccagctccaaacatcagcctcctcaggctgcagcccgacattctggagggctgttgaccctttcgagttctggaaaaatccctaaatcttatgttcaattaattaaaaatctatttgatttccatatcaggtgtccctgacagcagtcttccgtatcacttgctgccatatgaaaataatctttgaaaagttcataaagttcttcaaaaactggggccccccgtttctggaatcttcctgttgctctcttctcctttccagtttggcgtagaatgggttcttgagctgggttttttgttattgactttttttttttcctttttcttttttaaaataaaaaccatagatttcccaccctctttaatcccttccttttaaaaatgttctcttctctgctctacgtcctcccacttcccggttcaagtttcactggtgtcccgacccgtccccctgccctctgcccccccccccccccccgcccctgccccgtttgcattgtttgtgtgcggcatcttcagtataaaaggccagcgcccacggtcccaggagcgcctccctccttctctccctcctccctcgggccattctctccctccctccctccctccctcccctccagtgtttatatgtaagggtactggttgaccttggcggggctcagtgggtatccagtgtagacggtggaggctggcgaggcgctgatgtaggtctggtgggcaaattgggctggatactgactcgggtggatggtgggcgagggcaggacccgggggcccatgctcacggggacctggtggacgatgctggctgggtaggcagtgtgctgcacggtgtggcgcgcagagccttgcgaggccaccaggtgggccacggtgccggtggagcccagggccgccggcgcagtgtaggtgtagaggtggggctgggtggggaggtgggcagcggcagcggctgcagccagatgcgggtgcacagtgccgtggctggggctgttgtgcgggaaggagtacggagcctgggccatggtgggagtgatgtaggcctgctgccttcggtggctcccagtgcggtccgtggtgatgtgctgctgagcctggctgagattgagtggctgctgctgctggaagtgggggcccggccgctgctgccggtaggtgatggctccagatgagctccctgaagagtgaccgctggtggaggtcacgttgctggaggacttggacttgtaggaggacgagtggtgactggtgttgactggcaccaggctatcacactccaccaatacttcgctggcctgggttttcaggggtggcacgatgatggttcgggggttccccgtgcagtgattctccaggctccccttggtgtcaaaggcattggcattgttgtgcccagcacgctgctgcacggagtaggggctggtgttgctggaggagtcggagtagggggagtcgtggactgtgacacagctgatgacgttttttctttgcttggagacagtgctggtgggggcgtgtttctgttcctcctcctcgtccgtgtcactgctgatggtgatgacgctgaccgtggggctgggagtgtcgggaatgacaattgtctgccgctgccgttcccgggtggtgctggaggccacgtcgccccacccacaggtgaccgaggtgctgcaggccgggctactgtgcaccatggcacagcggggaggtgtgttctccttgacacgcttggatcgctgtggggagctgatggcctgagaggaggacacctcacaggtggagacatttctcacagatgactggtgctgcttactcttccgggaggaggtggtgctggttggctgctgccgcatcacgtgggccacacccacatttaagggctgtgctgctggaagggtcacatgaccggtcaatagtgcaggctgctgcatgatgggattataatggcttccgtgagcatgcgtatttctccagtccgccagctgctgggtgcctgccatggtctcgggaatcacggtggcatgctgcactgatgtgtgggtggccactccagtcagttgctgccatgctgggggaagcaggatctgctgggtcccacttggccaagcctgctgggcaagcagacctggttggatctgaagaggctgagctcctggggcttgagtgacgatgggaactgcattttccattcgcaccgagtagccagcgtgcttagagggagaggcctgcaagccttggaagccggggggacacacgatgagagcttgctggaacgggtcaggccgggcacaaatctgggctgttcctgtctgcaggggcatgctccgctgggccactgcagccatggatgccgctgagggctggtagagtgtagatgggtagtttagtatggagacttcgggattggctaaggaaatagtggcactggtagaggagggagcctggttgtggacagtggtcagctggttgttaaaggtcatggtcaggttggtggacgtgctgggggccacgtgcgtgatgaaaggggttttgctctggttcaccgtgtcatacatattcacccgacgcttgcagatctccatgttctggaaacatgatttgacgtgtgtgctgtggggaaaatcgagtaagtgtgtcatggtgacaaagggatggttcagggtttcgattggagtgattctcttgtcagcatcaatggtcagcatcttcttcaacaggtcaatgaactcccgccggtcagccttttctaccaacatgtcgctcccttccaaatctgtcgtcatgttcacctgggccatatcatctaaacagttgaaaatgtactttcttgcttcttttgacttaatccctgtctctgcttcatggtcatctggtgtcttcagtctccacaaaggatatggtgagtccgtgtcacggttgaaaaacctagttgtctttgtcccggcgcttaataaatattcagcaggcaaaccctgtgtttgtgaaatataccgaatctgatcatactccgaagctcctggatataacggccaacccaggaacaattctgcaataacacagcccagggaccacatgtcaattgcctcacaaaatggtaaaccaaggatgatctcaggggccctgtaatatctggactgcaagtaggtggagcacacagccttggagacgtggctggctgaaccaaagtcgatgaccttgactctgtatggttgtctagatggatccaccagcatgatgttttctggtttgaggtcagcgtggataagacctaggcttttgagtttcatcagggctgtggctacctgctggagaactgggcgaatgtatttgaggggcaaggggctaaacttgttttgcttcagaaagtcatagaggttctgctccaacatctcgaagaccaagcacgtgtggttcttgtgctggaagcattcgtaggcccggacgaagttatagtcatcggcactctccgtgctcaaccgggccaggatgctcacttcaatctgaccttgtcgggcataggatgggtggttcttcaggatcttgatggctacgatctcattggtgccccgtttccagcacttgaccacttgcccaaacgtccctcggcccaagaactctaagacctcgtaggtgttggtcatggagcacagcacctcatgctgcaccagctgatagtcgccctcgctgttggagccgctgtttttggaggtggcagtagacgtggtggcagtggcgacagtggccccgcttgcattattctgaatcatgggtggatgctcctcgatgatctgcacgctgcttgtgttctcgatctcctcgctcttacgcttgagtccacatttttggtaggtatcaaggaggctcacagtgcttcgacgcattaggttgtgtggtccgccgaggacttgcccggtgacagaagtgctgcttgctgaggtgaccacgatgtgcccggtgcttcctgggaagacgatggtctgctcgtaaggtaggcttgggtttgggaccggcaaggaggtgctgacggttgtggtggctggctgcgacagggggatgttcttgctctggctatacactttgctgtgggagccgtacccagtcatgtcccagttggaactcggctctattttcagtttcttcacactacagaaggcacttgattgaagggtgtgaggggagaaaacttgcacatgtgaggccataccttcgtacacgggggccatcggggccggggtgtccgcggttcatggcaacggggacgggaaagcggcgcgcgagctcggcccccccagcctcagtcggaatctgccatcttgagcctgtgtctccgctctcggcgcagccgaggccgcccgcgcccgcatcaccgcctcccgtggccggcgccgggggagggggccgggcgcgccgccgccgccgccgccgccgctgccgcccgggcccggcgcggggggctcggggctcggggctcggggcggccgggcgggcggagcggccgaggccgaggcgccgagcggccgcggcccccgagcggatccgcggaggggcgggagccgggggcagcgcgcggccagggccggcggggctcagctcagcat

SEQ ID NO: 16232 - RNA, 13762 nt, Homo sapiens
  source 1..13762: mol_type = other RNA
ggaggccggggtggggcggggcgggggtgtgctctctgttccatttgttagttacaggaagctaccaaggatgcacatggtcaagtcactttctacttcccaagttcctccttataacctgagccaaacaatttcaacaatgacaatccattgccccttcagcccagcaggcgactctgacagggaggtgtgaccaccagtctcaaggctgagtggggccttcttgctggctctcgcgctttctgggagtcctgggtgccttggcccagggcagtggtgacagcagggtggaggcagaggtggccccggggacagtgaccctatataaggaagggggcggtgccaggagagattcgtttggagattggttacaaggaagcgagggagagcagaggcagagccctttttcagatacaacatacttacttttcaaatgaacaaaaggcaatttctatgttttaaaaatataagccccaaaaacaatgacacaaaattcatttggttaattcatgtaaaggaaaaaacagcaacaccaccacacaaacaggaaagtgggagtatgattaggaggggtgagatgaaaactattttacagtaacatttccaccaaaagactgtcctaagaacacgctgtcaatacagttcacagggaaaaagcaaatgtggtatttttttgtattttttaaaagctccctggtcccaggtgttttgcagttttcaaggtcttatctgctaaaggaatgccctttaggtcacagcaggtcctctgcagtttggtggtggcacaagagaaaacataaaagaaaccaagactcagggaaactgccattcccccagtctgtttctgcatgacagtggggcccattcctgtctcgaagcatcttcttgttccaaatatgatgtctgtttagagtgggtctcaatggaccaggctgagctgcccctctgtctctgcctcctcctgctcagccctgaccatctctgagaggatgctaaggtccccctcccaccgaactagactttgagtctaagctggacaatgagtaaaacgtaaacatagccttttacattgattttgcttttaaggggaaaacgaataaatgacagcagatatatggaaaacccagccagcgaccatgggaataggggtatatggtcctcccctacaaaacgctgatcaaaatatcacccccggcccagaagtagcagctgtgccttcatggtcacctgaatcccagtctcttctactgcctggtgcctggaaatcagtggatctattaataagttaaatattcaaatcaagacaaaaatcaatgaaccaggttatctgttctcaatgactcttccaagatgtcagagagaaggccttgaagacaagtgtttagacgacacgcatgagaccttcgcatctggcccgggctgcggactcacaccttttccctccatctggattgcctttcatgttctcttgagttcacgtggaaagtaataatccagagggaagtgcgcatgctggactacagaagagtctgggacaacacacttgccttgggggagacacaacctccaactaagaggcattcactggggtttgcggatgtcagttataaacagaacttttctttaaaaagtaccagtctaaatgtaaactataaaacactttaactataaaacgtagccagaaatatgcttaagtatccacagtcaattgtttagtttactcatttaaaatgtgactgttttgatagcttagaaggctaacagcattttacagtagctaaaaacatatatacttaacatgtgcatttgaacatcgcatttgagtacaacacacaaagaataatctcttccttggtttaatttttgttgtaaagatgagctattttcagaattcacttaagcaacgatgaccgggggtatgaagtaatcattattttcagcccacagagaattcatagtctttaaattccaagatcaagctggctacatgatttcaaaaaaggctaaaaccaggatgaatgcccacatttgaggtaattattgccattaggtcacagtttgtgtaagataatgtatctaaaaccttctaaaaaaaaaaaaaatctttaggtgttctgccagaattccagaatacctattgaaaccaaccaggatctcaaactccgattagttaggtttgcttccaatggagttaaagttctaaaagattctagaacttgtgtaaactacctaagaatttaggcaaacaagcctggagccagtcaacaaagaaggttttaaatgaaaaaaggaacaagaaacccactcaaaacaactgaacaaatatttcataataaatgataatagttattttaaaaaattaaaaatctagtcctaagcatttctacattctcaccatctttcaatcaaaataaaaatgcatctgtatttctgttaatctcataccagggcaagagacacgccttccttttatcatgaaagctggctggttttcctgtttatacaattgttgctatttctttgagaagagtatctcaaaagaaaacattcttttgttcctctaagtcttgtctttcttccacctctacttctttttttttttcttttttttttcttttttttaacagaaagaaaaaagttcctggacaccagacccacatatggtatttacaaatttggtgtgaaccctgcctctggttctgcccagagctgaagagtgaatctattacagagatcagagctgtcaggataattatcaagtgcagtaaaaaatagcattttgaaaaaaatatatacctttagtattgcctttctagaattaactataagcaagaaaaacttattttttaaagaagaaaagaatactttttcactcttacttataagagctggttgtagcagcactactaaagctagttggtatgctggaaagaaatctaaaaggaattctatgaatcaaaagaaactctccagagattttctctaaaaatcaaacgaattctgccccttttgcctaaatccaactcaggagccccctctttgcacagtcctttagctgagtcccacggtgcatgggatggcacagggtgatgctgtgtaaaggcctttctttgctcagacatgcaggagacagctgtggctaatggctgcaagctcagttctggagctgggcagactcaggttcaagccctcctcgcccctcaagagttgtgtggctctgggcagtttccttggctgtagggggactaatattgccgatctcacagggctacggagaagatgaaacaggacaacccatgagcaattcccagcacagtgtgtggcatgcaggaagcgggagtatcactaaatggttcatagaaatatgaggccacgcattgctattaattaaaaaaagttaaaagattaaaaatcacatctcaggaagggcctgatgaacaaaaaagggaaccttggggattctggcccatcactgctttatccttccttcaacacctgccacttctcagagcatccggtcagctcccttatctataaatgggggctgttatccccctccctgtgggatggctgttggggccccttgagacaacgctcataaaggccttagcccgggagtcatgaaagcattcaacaaatgttggctattatttacttgagagatattgcaaattttaacaaataagggacagtcagtgtcatgttcaacacagggatctgagatgaggggctcccagaggcttgggcaagtccagcggggggcatcgggaagaccctctctggtgctggtgttctgggacgggagccctgcagggggcacttctctgcaaactctcactgggtttgagggaagaacggcctggagttcttttttgaacttttcagaagctgcaacaagagaaacctctactatgctgggtccctctagtgagccacggtgccaaaagcctccaataggttttttttgcatttaaatcctgtttcaccgccttccattctctagtggcctgagattttactgagtctggtctgtggagatgagaagtgagagttctaaggcatcaaagtggaaaagtactgctattccgagcccagcccccgcgtgctctacgcccttgatgcaactgaactcctggcagccctgctttgctctctcccatggtggcctgggattagtcaagcccacgtattggtatggcaccttgtctcccgatagcagcagcatcgaaggggtcacctccactcctcttaaaagaatagcacagttttgaaataaatgcattttttttttttaaaaaaaaggacagagaggaaagagaaagacaaatagaattgcatcactaatgatgtcattattgcctggaaaggaacgaagggaaggccattttgtccatttctggaggcgtctttgagaagggttctttggctaaagaaaggaacagtttcaccttcctttccaatttggtaaggacatctctggcctgctcaagtttgaagcttccccatcagaagtctgtaaaacacaccagaaggaaaagacacagacagggaatgaagcctgcaaagtccctggggctggaatgtcttgtggccaagtcactcctgctggcgctgtggagtcccaggctggcctgcagaaggaacccttacctctcctcaattctctctgctagttgagagcaccgagccatttccttctttccattttctgtcctagggtctacttgacaggccaacaagagtggtggtcccacaccccaccctgccctcagcatcagacaaagagaacctgggacaaaagctggggcgagctgggtccccacgtcgctctctcaaccatgagccatcagtaatacttcccgaagcctcctcatctcctccctccagtttccaagaaagtttgttccactcactcacacatgctcacacggcctaaatcttccaccccaagcttgttccaatatgagtgtttgccattcccaaggtccaaccaagggaaatcgttctgtcagcagttgggctaatctccccttcccttcctgatgtccatccgtctcacacgttggtgtctgggcgggctgagtcttctaggttgaagaggacaaaggtcagctggctcccccagcccgtgaacacctcagccaccaggaagactagaaaggctaacagtccaggagatgaatgccgctttgctccaacccttctttttcctctgaattccactgaccgcacgctccacttcacagtattaactggcatcaagcctcgactctcccaccccttgatctgctcacccacttcccttggaaacatccaaaacatcatgaagaggccctaagcacagagacatgggggcccacgtccagacgggccagtcagaacccagtgagcagaagcaaattgccctgcggttcaccaggctccagttaaacactcctccgtgacctgacatttcaaatcttcccctcttcctctgaacaatgtctcttcaaatgggaaggagggagcccacaaaagactagaggatgctctagatgattcgtgggctaagtaaggactaggttggcatccctctgcttgagagcttggtcctagtgacagcagcctatttgctaaggtgactcaatggcagattcggccaggtatgcaattgggcatccagggagctggcctctcctgcagggagcttctcttggggcttctgatgtggcagctccatgcatgggggtagaggaggccattgggtgaggactaggagaatgtgcactaatgtttgctgagcgtctgtggggctggcatcgcccaatacttcccttcccttcccttcggtgaagctggctatttcacccctttcttcaactggggcctagcactttgtgggtctggggacagcgtgtgagcacccagcgcacacagcacagtgcactgaagatgtggccggagcccagtggggatgctttcagagggggtgcagcctgtgatgcctgagcagccgcccagctttgttcagggtttctctggcctcctgctgtccctccacccacttccagctggctagaattgggtgctgggggcatgcatcacagggggagggggcaggctgaggaactgggtggtgtggtgaaatttcctggggaaggtaccacctgccagtcactcttacgccacctcactgtgcccagcagcttctgggagggggcaaatgtccctgcattgaagaacctaagccacgccccaggtgcgccgatggcaaaaggatggattgtggggaagcggatggggtcacctctgggagggaattttcttgcttaaataccagaggcaagccaaagatttagttaacagatttcagaagcacaggagagctctgaggatgtgggagagaagctggctaagggctggacagtcagtgactcgacattccccgagcccatgagatgccacctgacgtcgcatcccaggcctctgggatctagaaaatgacaaccttgatggtgaccatgttgtcagaagcccaatcaaggctttgattcttctttaaacttttgttctgtggtggatctttcttgacgtctcttgttgggatagagatgacagaaacaattttcctacttcctaagtctttcctttttttttttgcctgacaaaactggacatctggatgtccctccagtctacttatatactcacagagagaataagtttaaatattaaagagaaaacacaaagatacttggaataaatgtgcatttaaaaccctgactaaaatatcaacataatgatcataattacaatggtaataaaaataattagtacaataatattatctttatgagcagcatggaaatttcattcctgatctggaagaataaaaggaaagaaaatgtcaggtgaaagagtaagtagcctccaacttaagcagacagaataattttctttaaaatgaaaagaacattttaagctgtctttccccctaaaagatcagatctagaaagggctggaaatgaactgtgcccaggaatctgggggtgctctccagtaaggcgaactgaggctcatttgcagccaagacttggaactcgggatgagacctaatgggctattgctgccatctggctgccaaaaagtccctaatagatggattttccaggctgacccagctgtggggcgggggggggtcctctggcttctgtgtcctctgaagcgtttgctgccctcaccctctctgaactgaccattgtcctgctgtctcagagggctgcgcttccccacctccagataaagacagtattgataatggcccgagggaagggaatctccttgctgcaggcctcttgccggcacagcctccagcaggcacttggcaagactgcccggctgtgcccagcatggagcagtcatggtgtccttccttctcgctgaggcctggactaagctgtttccagtttggggacctgtttctttataagtaagaatttatggttggggtggggaagtttccagagttatttcacagctaagagctaagtaacgacttcgttactgagttaggttggatatcactacaaacacacctttcacagtagatccttgagggagactgcacagtgaggaagtaaagggagggaggatgaggatggggccgctgactcgggaaagatctctttgcaccttggaaacctgcctgtggggtcagctaaagactcaacatcagaagcaaacaattagaaccacccttttcggccccatccttggccagattctcctgccattcacattcacatatttcagagttatttactatgaagagagggaactccccacttctccacacctccatccccagaagtgtccaaagcctgagaaaacttccagaatgtatcaaaggtgcaaagagggcaaagggcagatttctttggaaattcaactgtgtgagtttttccaaagtgcagcgtcagacccccggccaccctcataagtgtccctccaaccttctgcccactagaaccctcagaaaccaaaaccaaaatcatgtcttgagcagacctgggtaatgtgaggagagaattcaacagcaaacagaggttggtggttgtctacagagggagggatctggcaagatcgttagagcaaaacagcccagggagccggaggagagagtggagccccgggcgaggctgagagctccaggctctcgtggaggcgggagggactgggggatgccgcctggggcgggagacggctgcctggcgaggccaacagtccggaaacctctggcctcacaaatggcggaactggggacagagtggggcaggggtgaagggtggggagtctctctgggcctccgcccacaaattacaactcaactactgccacaactcaactcccgccgtccccatctccagacgcacccgccgggcatctgtctcccatatttctttcgagatccacggactctctcctagctcctgctggcttccctggcatccttccgctagcaaacagcccaggaaagacaacgggcattaacattttaaaaagaaaaagaaaaagaaaaaaaaaaggccagcgtaaactgttacaacagcacaacagaagagctgagattgtgtctgactagcctcagtttcttggagtaccagtggaagtaaaccctcacgccgcgtctgtcgctcggtaaggcactaggagggaaggatgcagtgtcaagactgcgccagctagggtggcggcgccgagggccacgcggggagggcggcgcgtgcacacccacacgtgctcgctcacccgcacacctgcaccgccacattggttacatgcctatgttatatcgcttttttttgtgcaattacattgaggaatattctattggtatcattggagttgaacacaaggtaggagacaagggtgctgagtgctacattctactagggtgtctgtgacgaccgctagccctacgctacgcgactaggggtggattcaaagagaaaatacattttcagaaaagaaaaaaacctaaagtttgcaacacacattattaatgacatttgagaaacaacgttgcttagggatttatccagagtgctcagaaaaagaaaactcgccccgcgcccccgggggccttccagcagcctggccgtcccccgtctttcctgactagggagcccggactgggcttcgccaatcccacaccagctccaaacatcagcctcctcaggctgcagcccgacattctggagggctgttgaccctttcgagttctggaaaaatccctaaatcttatgttcaattaattaaaaatctatttgatttccatatcaggtgtccctgacagcagtcttccgtatcacttgctgccatatgaaaataatctttgaaaagttcataaagttcttcaaaaactggggccccccgtttctggaatcttcctgttgctctcttctcctttccagtttggcgtagaatgggttcttgagctgggttttttgttattgactttttttttttcctttttcttttttaaaataaaaaccatagatttcccaccctctttaatcccttccttttaaaaatgttctcttctctgctctacgtcctcccacttcccggttcaagtttcactggtgtcccgacccgtccccctgccctctgcccccccccccccccccgcccctgccccgtttgcattgtttgtgtgcggcatcttcagtataaaaggccagcgcccacggtcccaggagcgcctccctccttctctccctcctccctcgggccattctctccctccctccctccctccctcccctccagtgtttatatgtaagggtactggttgaccttggcggggctcagtgggtatccagtgtagacggtggaggctggcgaggcgctgatgtaggtctggtgggcaaattgggctggatactgactcgggtggatggtgggcgagggcaggacccgggggcccatgctcacggggacctggtggacgatgctggctgggtaggcagtgtgctgcacggtgtggcgcgcagagccttgcgaggccaccaggtgggccacggtgccggtggagcccagggccgccggcgcagtgtaggtgtagaggtggggctgggtggggaggtgggcagcggcagcggctgcagccagatgcgggtgcacagtgccgtggctggggctgttgtgcgggaaggagtacggagcctgggccatggtgggagtgatgtaggcctgctgccttcggtggctcccagtgcggtccgtggtgatgtgctgctgagcctggctgagattgagtggctgctgctgctggaagtgggggcccggccgctgctgccggtaggtgatggctccagatgagctccctgaagagtgaccgctggtggaggtcacgttgctggaggacttggacttgtaggaggacgagtggtgactggtgttgactggcaccaggctatcacactccaccaatacttcgctggcctgggttttcaggggtggcacgatgatggttcgggggttccccgtgcagtgattctccaggctccccttggtgtcaaaggcattggcattgttgtgcccagcacgctgctgcacggagtaggggctggtgttgctggaggagtcggagtagggggagtcgtggactgtgacacagctgatgacgttttttctttgcttggagacagtgctggtgggggcgtgtttctgttcctcctcctcgtccgtgtcactgctgatggtgatgacgctgaccgtggggctgggagtgtcgggaatgacaattgtctgccgctgccgttcccgggtggtgctggaggccacgtcgccccacccacaggtgaccgaggtgctgcaggccgggctactgtgcaccatggcacagcggggaggtgtgttctccttgacacgcttggatcgctgtggggagctgatggcctgagaggaggacacctcacaggtggagacatttctcacagatgactggtgctgcttactcttccgggaggaggtggtgctggttggctgctgccgcatcacgtgggccacacccacatttaagggctgtgctgctggaagggtcacatgaccggtcaatagtgcaggctgctgcatgatgggattataatggcttccgtgagcatgcgtatttctccagtccgccagctgctgggtgcctgccatggtctcgggaatcacggtggcatgctgcactgatgtgtgggtggccactccagtcagttgctgccatgctgggggaagcaggatctgctgggtcccacttggccaagcctgctgggcaagcagacctggttggatctgaagaggctgagctcctggggcttgagtgacgatgggaactgcattttccattcgcaccgagtagccagcgtgcttagagggagaggcctgcaagccttggaagccggggggacacacgatgagagcttgctggaacgggtcaggccgggcacaaatctgggctgttcctgtctgcaggggcatgctccgctgggccactgcagccatggatgccgctgagggctggtagagtgtagatgggtagtttagtatggagacttcgggattggctaaggaaatagtggcactggtagaggagggagcctggttgtggacagtggtcagctggttgttaaaggtcatggtcaggttggtggacgtgctgggggccacgtgcgtgatgaaaggggttttgctctggttcaccgtgtcatacatattcacccgacgcttgcagatctccatgttctggaaacatgatttgacgtgtgtgctgtggggaaaatcgagtaagtgtgtcatggtgacaaagggatggttcagggtttcgattggagtgattctcttgtcagcatcaatggtcagcatcttcttcaacaggtcaatgaactcccgccggtcagccttttctaccaacatgtcgctcccttccaaatctgtcgtcatgttcacctgggccatatcatctaaacagttgaaaatgtactttcttgcttcttttgacttaatccctgtctctgcttcatggtcatctggtgtcttcagtctccacaaaggatatggtgagtccgtgtcacggttgaaaaacctagttgtctttgtcccggcgcttaataaatattcagcaggcaaaccctgtgtttgtgaaatataccgaatctgatcatactccgaagctcctggatataacggccaacccaggaacaattctgcaataacacagcccagggaccacatgtcaattgcctcacaaaatggtaaaccaaggatgatctcaggggccctgtaatatctggactgcaagtaggtggagcacacagccttggagacgtggctggctgaaccaaagtcgatgaccttgactctgtatggttgtctagatggatccaccagcatgatgttttctggtttgaggtcagcgtggataagacctaggcttttgagtttcatcagggctgtggctacctgctggagaactgggcgaatgtatttgaggggcaaggggctaaacttgttttgcttcagaaagtcatagaggttctgctccaacatctcgaagaccaagcacgtgtggttcttgtgctggaagcattcgtaggcccggacgaagttatagtcatcggcactctccgtgctcaaccgggccaggatgctcacttcaatctgaccttgtcgggcataggatgggtggttcttcaggatcttgatggctacgatctcattggtgccccgtttccagcacttgaccacttgcccaaacgtccctcggcccaagaactctaagacctcgtaggtgttggtcatggagcacagcacctcatgctgcaccagctgatagtcgccctcgctgttggagccgctgtttttggaggtggcagtagacgtggtggcagtggcgacagtggccccgcttgcattattctgaatcatgggtggatgctcctcgatgatctgcacgctgcttgtgttctcgatctcctcgctcttacgcttgagtccacatttttggtaggtatcaaggaggctcacagtgcttcgacgcattaggttgtgtggtccgccgaggacttgcccggtgacagaagtgctgcttgctgaggtgaccacgatgtgcccggtgcttcctgggaagacgatggtctgctcgtaaggtaggcttgggtttgggaccggcaaggaggtgctgacggttgtggtggctggctgcgacagggggatgttcttgctctggctatacactttgctgtgggagccgtacccagtcatgtcccagttggaactcggctctattttcagtttcttcacactacagaaggcacttgattgaagggtgtgaggggagaaaacttgcacatgtgaggccatacctttgttatttctccaattccgtgaacgttgatcagttcagtatagctctgaattttcacaggtaactcctcctgtctcctgtgcattcattttctcagtcactattcaataaatactcagtatgatcaccaccattcacgttttgttgtttgtaatatggttcgtcttttgaaatcatagataagtggcacagaacctggtatgatgaaaaatgtcagagaaaacaaagataagaacgtgaacttgatctttacatacactctctcatctaagcctcacggcaaccctgggaggtcattattatcatcctcaccttacagaagaaagagatccagagagactggcaggattcgctcccccaaggtcatga

SEQ ID NO: 16233 - RNA, 13670 nt, Homo sapiens
  source 1..13670: mol_type = other RNA
ggaggccggggtggggcggggcgggggtgtgctctctgttccatttgttagttacaggaagctaccaaggatgcacatggtcaagtcactttctacttcccaagttcctccttataacctgagccaaacaatttcaacaatgacaatccattgccccttcagcccagcaggcgactctgacagggaggtgtgaccaccagtctcaaggctgagtggggccttcttgctggctctcgcgctttctgggagtcctgggtgccttggcccagggcagtggtgacagcagggtggaggcagaggtggccccggggacagtgaccctatataaggaagggggcggtgccaggagagattcgtttggagattggttacaaggaagcgagggagagcagaggcagagccctttttcagatacaacatacttacttttcaaatgaacaaaaggcaatttctatgttttaaaaatataagccccaaaaacaatgacacaaaattcatttggttaattcatgtaaaggaaaaaacagcaacaccaccacacaaacaggaaagtgggagtatgattaggaggggtgagatgaaaactattttacagtaacatttccaccaaaagactgtcctaagaacacgctgtcaatacagttcacagggaaaaagcaaatgtggtatttttttgtattttttaaaagctccctggtcccaggtgttttgcagttttcaaggtcttatctgctaaaggaatgccctttaggtcacagcaggtcctctgcagtttggtggtggcacaagagaaaacataaaagaaaccaagactcagggaaactgccattcccccagtctgtttctgcatgacagtggggcccattcctgtctcgaagcatcttcttgttccaaatatgatgtctgtttagagtgggtctcaatggaccaggctgagctgcccctctgtctctgcctcctcctgctcagccctgaccatctctgagaggatgctaaggtccccctcccaccgaactagactttgagtctaagctggacaatgagtaaaacgtaaacatagccttttacattgattttgcttttaaggggaaaacgaataaatgacagcagatatatggaaaacccagccagcgaccatgggaataggggtatatggtcctcccctacaaaacgctgatcaaaatatcacccccggcccagaagtagcagctgtgccttcatggtcacctgaatcccagtctcttctactgcctggtgcctggaaatcagtggatctattaataagttaaatattcaaatcaagacaaaaatcaatgaaccaggttatctgttctcaatgactcttccaagatgtcagagagaaggccttgaagacaagtgtttagacgacacgcatgagaccttcgcatctggcccgggctgcggactcacaccttttccctccatctggattgcctttcatgttctcttgagttcacgtggaaagtaataatccagagggaagtgcgcatgctggactacagaagagtctgggacaacacacttgccttgggggagacacaacctccaactaagaggcattcactggggtttgcggatgtcagttataaacagaacttttctttaaaaagtaccagtctaaatgtaaactataaaacactttaactataaaacgtagccagaaatatgcttaagtatccacagtcaattgtttagtttactcatttaaaatgtgactgttttgatagcttagaaggctaacagcattttacagtagctaaaaacatatatacttaacatgtgcatttgaacatcgcatttgagtacaacacacaaagaataatctcttccttggtttaatttttgttgtaaagatgagctattttcagaattcacttaagcaacgatgaccgggggtatgaagtaatcattattttcagcccacagagaattcatagtctttaaattccaagatcaagctggctacatgatttcaaaaaaggctaaaaccaggatgaatgcccacatttgaggtaattattgccattaggtcacagtttgtgtaagataatgtatctaaaaccttctaaaaaaaaaaaaaatctttaggtgttctgccagaattccagaatacctattgaaaccaaccaggatctcaaactccgattagttaggtttgcttccaatggagttaaagttctaaaagattctagaacttgtgtaaactacctaagaatttaggcaaacaagcctggagccagtcaacaaagaaggttttaaatgaaaaaaggaacaagaaacccactcaaaacaactgaacaaatatttcataataaatgataatagttattttaaaaaattaaaaatctagtcctaagcatttctacattctcaccatctttcaatcaaaataaaaatgcatctgtatttctgttaatctcataccagggcaagagacacgccttccttttatcatgaaagctggctggttttcctgtttatacaattgttgctatttctttgagaagagtatctcaaaagaaaacattcttttgttcctctaagtcttgtctttcttccacctctacttctttttttttttcttttttttttcttttttttaacagaaagaaaaaagttcctggacaccagacccacatatggtatttacaaatttggtgtgaaccctgcctctggttctgcccagagctgaagagtgaatctattacagagatcagagctgtcaggataattatcaagtgcagtaaaaaatagcattttgaaaaaaatatatacctttagtattgcctttctagaattaactataagcaagaaaaacttattttttaaagaagaaaagaatactttttcactcttacttataagagctggttgtagcagcactactaaagctagttggtatgctggaaagaaatctaaaaggaattctatgaatcaaaagaaactctccagagattttctctaaaaatcaaacgaattctgccccttttgcctaaatccaactcaggagccccctctttgcacagtcctttagctgagtcccacggtgcatgggatggcacagggtgatgctgtgtaaaggcctttctttgctcagacatgcaggagacagctgtggctaatggctgcaagctcagttctggagctgggcagactcaggttcaagccctcctcgcccctcaagagttgtgtggctctgggcagtttccttggctgtagggggactaatattgccgatctcacagggctacggagaagatgaaacaggacaacccatgagcaattcccagcacagtgtgtggcatgcaggaagcgggagtatcactaaatggttcatagaaatatgaggccacgcattgctattaattaaaaaaagttaaaagattaaaaatcacatctcaggaagggcctgatgaacaaaaaagggaaccttggggattctggcccatcactgctttatccttccttcaacacctgccacttctcagagcatccggtcagctcccttatctataaatgggggctgttatccccctccctgtgggatggctgttggggccccttgagacaacgctcataaaggccttagcccgggagtcatgaaagcattcaacaaatgttggctattatttacttgagagatattgcaaattttaacaaataagggacagtcagtgtcatgttcaacacagggatctgagatgaggggctcccagaggcttgggcaagtccagcggggggcatcgggaagaccctctctggtgctggtgttctgggacgggagccctgcagggggcacttctctgcaaactctcactgggtttgagggaagaacggcctggagttcttttttgaacttttcagaagctgcaacaagagaaacctctactatgctgggtccctctagtgagccacggtgccaaaagcctccaataggttttttttgcatttaaatcctgtttcaccgccttccattctctagtggcctgagattttactgagtctggtctgtggagatgagaagtgagagttctaaggcatcaaagtggaaaagtactgctattccgagcccagcccccgcgtgctctacgcccttgatgcaactgaactcctggcagccctgctttgctctctcccatggtggcctgggattagtcaagcccacgtattggtatggcaccttgtctcccgatagcagcagcatcgaaggggtcacctccactcctcttaaaagaatagcacagttttgaaataaatgcattttttttttttaaaaaaaaggacagagaggaaagagaaagacaaatagaattgcatcactaatgatgtcattattgcctggaaaggaacgaagggaaggccattttgtccatttctggaggcgtctttgagaagggttctttggctaaagaaaggaacagtttcaccttcctttccaatttggtaaggacatctctggcctgctcaagtttgaagcttccccatcagaagtctgtaaaacacaccagaaggaaaagacacagacagggaatgaagcctgcaaagtccctggggctggaatgtcttgtggccaagtcactcctgctggcgctgtggagtcccaggctggcctgcagaaggaacccttacctctcctcaattctctctgctagttgagagcaccgagccatttccttctttccattttctgtcctagggtctacttgacaggccaacaagagtggtggtcccacaccccaccctgccctcagcatcagacaaagagaacctgggacaaaagctggggcgagctgggtccccacgtcgctctctcaaccatgagccatcagtaatacttcccgaagcctcctcatctcctccctccagtttccaagaaagtttgttccactcactcacacatgctcacacggcctaaatcttccaccccaagcttgttccaatatgagtgtttgccattcccaaggtccaaccaagggaaatcgttctgtcagcagttgggctaatctccccttcccttcctgatgtccatccgtctcacacgttggtgtctgggcgggctgagtcttctaggttgaagaggacaaaggtcagctggctcccccagcccgtgaacacctcagccaccaggaagactagaaaggctaacagtccaggagatgaatgccgctttgctccaacccttctttttcctctgaattccactgaccgcacgctccacttcacagtattaactggcatcaagcctcgactctcccaccccttgatctgctcacccacttcccttggaaacatccaaaacatcatgaagaggccctaagcacagagacatgggggcccacgtccagacgggccagtcagaacccagtgagcagaagcaaattgccctgcggttcaccaggctccagttaaacactcctccgtgacctgacatttcaaatcttcccctcttcctctgaacaatgtctcttcaaatgggaaggagggagcccacaaaagactagaggatgctctagatgattcgtgggctaagtaaggactaggttggcatccctctgcttgagagcttggtcctagtgacagcagcctatttgctaaggtgactcaatggcagattcggccaggtatgcaattgggcatccagggagctggcctctcctgcagggagcttctcttggggcttctgatgtggcagctccatgcatgggggtagaggaggccattgggtgaggactaggagaatgtgcactaatgtttgctgagcgtctgtggggctggcatcgcccaatacttcccttcccttcccttcggtgaagctggctatttcacccctttcttcaactggggcctagcactttgtgggtctggggacagcgtgtgagcacccagcgcacacagcacagtgcactgaagatgtggccggagcccagtggggatgctttcagagggggtgcagcctgtgatgcctgagcagccgcccagctttgttcagggtttctctggcctcctgctgtccctccacccacttccagctggctagaattgggtgctgggggcatgcatcacagggggagggggcaggctgaggaactgggtggtgtggtgaaatttcctggggaaggtaccacctgccagtcactcttacgccacctcactgtgcccagcagcttctgggagggggcaaatgtccctgcattgaagaacctaagccacgccccaggtgcgccgatggcaaaaggatggattgtggggaagcggatggggtcacctctgggagggaattttcttgcttaaataccagaggcaagccaaagatttagttaacagatttcagaagcacaggagagctctgaggatgtgggagagaagctggctaagggctggacagtcagtgactcgacattccccgagcccatgagatgccacctgacgtcgcatcccaggcctctgggatctagaaaatgacaaccttgatggtgaccatgttgtcagaagcccaatcaaggctttgattcttctttaaacttttgttctgtggtggatctttcttgacgtctcttgttgggatagagatgacagaaacaattttcctacttcctaagtctttcctttttttttttgcctgacaaaactggacatctggatgtccctccagtctacttatatactcacagagagaataagtttaaatattaaagagaaaacacaaagatacttggaataaatgtgcatttaaaaccctgactaaaatatcaacataatgatcataattacaatggtaataaaaataattagtacaataatattatctttatgagcagcatggaaatttcattcctgatctggaagaataaaaggaaagaaaatgtcaggtgaaagagtaagtagcctccaacttaagcagacagaataattttctttaaaatgaaaagaacattttaagctgtctttccccctaaaagatcagatctagaaagggctggaaatgaactgtgcccaggaatctgggggtgctctccagtaaggcgaactgaggctcatttgcagccaagacttggaactcgggatgagacctaatgggctattgctgccatctggctgccaaaaagtccctaatagatggattttccaggctgacccagctgtggggcgggggggggtcctctggcttctgtgtcctctgaagcgtttgctgccctcaccctctctgaactgaccattgtcctgctgtctcagagggctgcgcttccccacctccagataaagacagtattgataatggcccgagggaagggaatctccttgctgcaggcctcttgccggcacagcctccagcaggcacttggcaagactgcccggctgtgcccagcatggagcagtcatggtgtccttccttctcgctgaggcctggactaagctgtttccagtttggggacctgtttctttataagtaagaatttatggttggggtggggaagtttccagagttatttcacagctaagagctaagtaacgacttcgttactgagttaggttggatatcactacaaacacacctttcacagtagatccttgagggagactgcacagtgaggaagtaaagggagggaggatgaggatggggccgctgactcgggaaagatctctttgcaccttggaaacctgcctgtggggtcagctaaagactcaacatcagaagcaaacaattagaaccacccttttcggccccatccttggccagattctcctgccattcacattcacatatttcagagttatttactatgaagagagggaactccccacttctccacacctccatccccagaagtgtccaaagcctgagaaaacttccagaatgtatcaaaggtgcaaagagggcaaagggcagatttctttggaaattcaactgtgtgagtttttccaaagtgcagcgtcagacccccggccaccctcataagtgtccctccaaccttctgcccactagaaccctcagaaaccaaaaccaaaatcatgtcttgagcagacctgggtaatgtgaggagagaattcaacagcaaacagaggttggtggttgtctacagagggagggatctggcaagatcgttagagcaaaacagcccagggagccggaggagagagtggagccccgggcgaggctgagagctccaggctctcgtggaggcgggagggactgggggatgccgcctggggcgggagacggctgcctggcgaggccaacagtccggaaacctctggcctcacaaatggcggaactggggacagagtggggcaggggtgaagggtggggagtctctctgggcctccgcccacaaattacaactcaactactgccacaactcaactcccgccgtccccatctccagacgcacccgccgggcatctgtctcccatatttctttcgagatccacggactctctcctagctcctgctggcttccctggcatccttccgctagcaaacagcccaggaaagacaacgggcattaacattttaaaaagaaaaagaaaaagaaaaaaaaaaggccagcgtaaactgttacaacagcacaacagaagagctgagattgtgtctgactagcctcagtttcttggagtaccagtggaagtaaaccctcacgccgcgtctgtcgctcggtaaggcactaggagggaaggatgcagtgtcaagactgcgccagctagggtggcggcgccgagggccacgcggggagggcggcgcgtgcacacccacacgtgctcgctcacccgcacacctgcaccgccacattggttacatgcctatgttatatcgcttttttttgtgcaattacattgaggaatattctattggtatcattggagttgaacacaaggtaggagacaagggtgctgagtgctacattctactagggtgtctgtgacgaccgctagccctacgctacgcgactaggggtggattcaaagagaaaatacattttcagaaaagaaaaaaacctaaagtttgcaacacacattattaatgacatttgagaaacaacgttgcttagggatttatccagagtgctcagaaaaagaaaactcgccccgcgcccccgggggccttccagcagcctggccgtcccccgtctttcctgactagggagcccggactgggcttcgccaatcccacaccagctccaaacatcagcctcctcaggctgcagcccgacattctggagggctgttgaccctttcgagttctggaaaaatccctaaatcttatgttcaattaattaaaaatctatttgatttccatatcaggtgtccctgacagcagtcttccgtatcacttgctgccatatgaaaataatctttgaaaagttcataaagttcttcaaaaactggggccccccgtttctggaatcttcctgttgctctcttctcctttccagtttggcgtagaatgggttcttgagctgggttttttgttattgactttttttttttcctttttcttttttaaaataaaaaccatagatttcccaccctctttaatcccttccttttaaaaatgttctcttctctgctctacgtcctcccacttcccggttcaagtttcactggtgtcccgacccgtccccctgccctctgcccccccccccccccccgcccctgccccgtttgcattgtttgtgtgcggcatcttcagtataaaaggccagcgcccacggtcccaggagcgcctccctccttctctccctcctccctcgggccattctctccctccctccctccctccctcccctccagtgtttatatgtaagggtactggttgaccttggcggggctcagtgggtatccagtgtagacggtggaggctggcgaggcgctgatgtaggtctggtgggcaaattgggctggatactgactcgggtggatggtgggcgagggcaggacccgggggcccatgctcacggggacctggtggacgatgctggctgggtaggcagtgtgctgcacggtgtggcgcgcagagccttgcgaggccaccaggtgggccacggtgccggtggagcccagggccgccggcgcagtgtaggtgtagaggtggggctgggtggggaggtgggcagcggcagcggctgcagccagatgcgggtgcacagtgccgtggctggggctgttgtgcgggaaggagtacggagcctgggccatggtgggagtgatgtaggcctgctgccttcggtggctcccagtgcggtccgtggtgatgtgctgctgagcctggctgagattgagtggctgctgctgctggaagtgggggcccggccgctgctgccggtaggtgatggctccagatgagctccctgaagagtgaccgctggtggaggtcacgttgctggaggacttggacttgtaggaggacgagtggtgactggtgttgactggcaccaggctatcacactccaccaatacttcgctggcctgggttttcaggggtggcacgatgatggttcgggggttccccgtgcagtgattctccaggctccccttggtgtcaaaggcattggcattgttgtgcccagcacgctgctgcacggagtaggggctggtgttgctggaggagtcggagtagggggagtcgtggactgtgacacagctgatgacgttttttctttgcttggagacagtgctggtgggggcgtgtttctgttcctcctcctcgtccgtgtcactgctgatggtgatgacgctgaccgtggggctgggagtgtcgggaatgacaattgtctgccgctgccgttcccgggtggtgctggaggccacgtcgccccacccacaggtgaccgaggtgctgcaggccgggctactgtgcaccatggcacagcggggaggtgtgttctccttgacacgcttggatcgctgtggggagctgatggcctgagaggaggacacctcacaggtggagacatttctcacagatgactggtgctgcttactcttccgggaggaggtggtgctggttggctgctgccgcatcacgtgggccacacccacatttaagggctgtgctgctggaagggtcacatgaccggtcaatagtgcaggctgctgcatgatgggattataatggcttccgtgagcatgcgtatttctccagtccgccagctgctgggtgcctgccatggtctcgggaatcacggtggcatgctgcactgatgtgtgggtggccactccagtcagttgctgccatgctgggggaagcaggatctgctgggtcccacttggccaagcctgctgggcaagcagacctggttggatctgaagaggctgagctcctggggcttgagtgacgatgggaactgcattttccattcgcaccgagtagccagcgtgcttagagggagaggcctgcaagccttggaagccggggggacacacgatgagagcttgctggaacgggtcaggccgggcacaaatctgggctgttcctgtctgcaggggcatgctccgctgggccactgcagccatggatgccgctgagggctggtagagtgtagatgggtagtttagtatggagacttcgggattggctaaggaaatagtggcactggtagaggagggagcctggttgtggacagtggtcagctggttgttaaaggtcatggtcaggttggtggacgtgctgggggccacgtgcgtgatgaaaggggttttgctctggttcaccgtgtcatacatattcacccgacgcttgcagatctccatgttctggaaacatgatttgacgtgtgtgctgtggggaaaatcgagtaagtgtgtcatggtgacaaagggatggttcagggtttcgattggagtgattctcttgtcagcatcaatggtcagcatcttcttcaacaggtcaatgaactcccgccggtcagccttttctaccaacatgtcgctcccttccaaatctgtcgtcatgttcacctgggccatatcatctaaacagttgaaaatgtactttcttgcttcttttgacttaatccctgtctctgcttcatggtcatctggtgtcttcagtctccacaaaggatatggtgagtccgtgtcacggttgaaaaacctagttgtctttgtcccggcgcttaataaatattcagcaggcaaaccctgtgtttgtgaaatataccgaatctgatcatactccgaagctcctggatataacggccaacccaggaacaattctgcaataacacagcccagggaccacatgtcaattgcctcacaaaatggtaaaccaaggatgatctcaggggccctgtaatatctggactgcaagtaggtggagcacacagccttggagacgtggctggctgaaccaaagtcgatgaccttgactctgtatggttgtctagatggatccaccagcatgatgttttctggtttgaggtcagcgtggataagacctaggcttttgagtttcatcagggctgtggctacctgctggagaactgggcgaatgtatttgaggggcaaggggctaaacttgttttgcttcagaaagtcatagaggttctgctccaacatctcgaagaccaagcacgtgtggttcttgtgctggaagcattcgtaggcccggacgaagttatagtcatcggcactctccgtgctcaaccgggccaggatgctcacttcaatctgaccttgtcgggcataggatgggtggttcttcaggatcttgatggctacgatctcattggtgccccgtttccagcacttgaccacttgcccaaacgtccctcggcccaagaactctaagacctcgtaggtgttggtcatggagcacagcacctcatgctgcaccagctgatagtcgccctcgctgttggagccgctgtttttggaggtggcagtagacgtggtggcagtggcgacagtggccccgcttgcattattctgaatcatgggtggatgctcctcgatgatctgcacgctgcttgtgttctcgatctcctcgctcttacgcttgagtccacatttttggtaggtatcaaggaggctcacagtgcttcgacgcattaggttgtgtggtccgccgaggacttgcccggtgacagaagtgctgcttgctgaggtgaccacgatgtgcccggtgcttcctgggaagacgatggtctgctcgtaaggtaggcttgggtttgggaccggcaaggaggtgctgacggttgtggtggctggctgcgacagggggatgttcttgctctggctatacactttgctgtgggagccgtacccagtcatgtcccagttggaactcggctctattttcagtttcttcacactacagaaggcacttgattgaagggtgtgaggggagaaaacttgcacatgtgaggccatacctttgttatttctccaattccgtgaacgttgatcagttcagtatagctctgaattttcacaggtaactcctcctgtctcctgtgcattcattttctcagtcactattcaataaatactcagtatgatcaccaccattcacgttttgttgtttgtaatatggttcgtcttttgaaatcatagataagtggcacagaaccttacagaagaaagagatccagagagactggcaggattcgctcccccaaggtcatgagctcgtaaaatcagaggacctgaat

SEQ ID NO: 16234 - RNA, 14177 nt, Homo sapiens
  source 1..14177: mol_type = other RNA
ggaggccggggtggggcggggcgggggtgtgctctctgttccatttgttagttacaggaagctaccaaggatgcacatggtcaagtcactttctacttcccaagttcctccttataacctgagccaaacaatttcaacaatgacaatccattgccccttcagcccagcaggcgactctgacagggaggtgtgaccaccagtctcaaggctgagtggggccttcttgctggctctcgcgctttctgggagtcctgggtgccttggcccagggcagtggtgacagcagggtggaggcagaggtggccccggggacagtgaccctatataaggaagggggcggtgccaggagagattcgtttggagattggttacaaggaagcgagggagagcagaggcagagccctttttcagatacaacatacttacttttcaaatgaacaaaaggcaatttctatgttttaaaaatataagccccaaaaacaatgacacaaaattcatttggttaattcatgtaaaggaaaaaacagcaacaccaccacacaaacaggaaagtgggagtatgattaggaggggtgagatgaaaactattttacagtaacatttccaccaaaagactgtcctaagaacacgctgtcaatacagttcacagggaaaaagcaaatgtggtatttttttgtattttttaaaagctccctggtcccaggtgttttgcagttttcaaggtcttatctgctaaaggaatgccctttaggtcacagcaggtcctctgcagtttggtggtggcacaagagaaaacataaaagaaaccaagactcagggaaactgccattcccccagtctgtttctgcatgacagtggggcccattcctgtctcgaagcatcttcttgttccaaatatgatgtctgtttagagtgggtctcaatggaccaggctgagctgcccctctgtctctgcctcctcctgctcagccctgaccatctctgagaggatgctaaggtccccctcccaccgaactagactttgagtctaagctggacaatgagtaaaacgtaaacatagccttttacattgattttgcttttaaggggaaaacgaataaatgacagcagatatatggaaaacccagccagcgaccatgggaataggggtatatggtcctcccctacaaaacgctgatcaaaatatcacccccggcccagaagtagcagctgtgccttcatggtcacctgaatcccagtctcttctactgcctggtgcctggaaatcagtggatctattaataagttaaatattcaaatcaagacaaaaatcaatgaaccaggttatctgttctcaatgactcttccaagatgtcagagagaaggccttgaagacaagtgtttagacgacacgcatgagaccttcgcatctggcccgggctgcggactcacaccttttccctccatctggattgcctttcatgttctcttgagttcacgtggaaagtaataatccagagggaagtgcgcatgctggactacagaagagtctgggacaacacacttgccttgggggagacacaacctccaactaagaggcattcactggggtttgcggatgtcagttataaacagaacttttctttaaaaagtaccagtctaaatgtaaactataaaacactttaactataaaacgtagccagaaatatgcttaagtatccacagtcaattgtttagtttactcatttaaaatgtgactgttttgatagcttagaaggctaacagcattttacagtagctaaaaacatatatacttaacatgtgcatttgaacatcgcatttgagtacaacacacaaagaataatctcttccttggtttaatttttgttgtaaagatgagctattttcagaattcacttaagcaacgatgaccgggggtatgaagtaatcattattttcagcccacagagaattcatagtctttaaattccaagatcaagctggctacatgatttcaaaaaaggctaaaaccaggatgaatgcccacatttgaggtaattattgccattaggtcacagtttgtgtaagataatgtatctaaaaccttctaaaaaaaaaaaaaatctttaggtgttctgccagaattccagaatacctattgaaaccaaccaggatctcaaactccgattagttaggtttgcttccaatggagttaaagttctaaaagattctagaacttgtgtaaactacctaagaatttaggcaaacaagcctggagccagtcaacaaagaaggttttaaatgaaaaaaggaacaagaaacccactcaaaacaactgaacaaatatttcataataaatgataatagttattttaaaaaattaaaaatctagtcctaagcatttctacattctcaccatctttcaatcaaaataaaaatgcatctgtatttctgttaatctcataccagggcaagagacacgccttccttttatcatgaaagctggctggttttcctgtttatacaattgttgctatttctttgagaagagtatctcaaaagaaaacattcttttgttcctctaagtcttgtctttcttccacctctacttctttttttttttcttttttttttcttttttttaacagaaagaaaaaagttcctggacaccagacccacatatggtatttacaaatttggtgtgaaccctgcctctggttctgcccagagctgaagagtgaatctattacagagatcagagctgtcaggataattatcaagtgcagtaaaaaatagcattttgaaaaaaatatatacctttagtattgcctttctagaattaactataagcaagaaaaacttattttttaaagaagaaaagaatactttttcactcttacttataagagctggttgtagcagcactactaaagctagttggtatgctggaaagaaatctaaaaggaattctatgaatcaaaagaaactctccagagattttctctaaaaatcaaacgaattctgccccttttgcctaaatccaactcaggagccccctctttgcacagtcctttagctgagtcccacggtgcatgggatggcacagggtgatgctgtgtaaaggcctttctttgctcagacatgcaggagacagctgtggctaatggctgcaagctcagttctggagctgggcagactcaggttcaagccctcctcgcccctcaagagttgtgtggctctgggcagtttccttggctgtagggggactaatattgccgatctcacagggctacggagaagatgaaacaggacaacccatgagcaattcccagcacagtgtgtggcatgcaggaagcgggagtatcactaaatggttcatagaaatatgaggccacgcattgctattaattaaaaaaagttaaaagattaaaaatcacatctcaggaagggcctgatgaacaaaaaagggaaccttggggattctggcccatcactgctttatccttccttcaacacctgccacttctcagagcatccggtcagctcccttatctataaatgggggctgttatccccctccctgtgggatggctgttggggccccttgagacaacgctcataaaggccttagcccgggagtcatgaaagcattcaacaaatgttggctattatttacttgagagatattgcaaattttaacaaataagggacagtcagtgtcatgttcaacacagggatctgagatgaggggctcccagaggcttgggcaagtccagcggggggcatcgggaagaccctctctggtgctggtgttctgggacgggagccctgcagggggcacttctctgcaaactctcactgggtttgagggaagaacggcctggagttcttttttgaacttttcagaagctgcaacaagagaaacctctactatgctgggtccctctagtgagccacggtgccaaaagcctccaataggttttttttgcatttaaatcctgtttcaccgccttccattctctagtggcctgagattttactgagtctggtctgtggagatgagaagtgagagttctaaggcatcaaagtggaaaagtactgctattccgagcccagcccccgcgtgctctacgcccttgatgcaactgaactcctggcagccctgctttgctctctcccatggtggcctgggattagtcaagcccacgtattggtatggcaccttgtctcccgatagcagcagcatcgaaggggtcacctccactcctcttaaaagaatagcacagttttgaaataaatgcattttttttttttaaaaaaaaggacagagaggaaagagaaagacaaatagaattgcatcactaatgatgtcattattgcctggaaaggaacgaagggaaggccattttgtccatttctggaggcgtctttgagaagggttctttggctaaagaaaggaacagtttcaccttcctttccaatttggtaaggacatctctggcctgctcaagtttgaagcttccccatcagaagtctgtaaaacacaccagaaggaaaagacacagacagggaatgaagcctgcaaagtccctggggctggaatgtcttgtggccaagtcactcctgctggcgctgtggagtcccaggctggcctgcagaaggaacccttacctctcctcaattctctctgctagttgagagcaccgagccatttccttctttccattttctgtcctagggtctacttgacaggccaacaagagtggtggtcccacaccccaccctgccctcagcatcagacaaagagaacctgggacaaaagctggggcgagctgggtccccacgtcgctctctcaaccatgagccatcagtaatacttcccgaagcctcctcatctcctccctccagtttccaagaaagtttgttccactcactcacacatgctcacacggcctaaatcttccaccccaagcttgttccaatatgagtgtttgccattcccaaggtccaaccaagggaaatcgttctgtcagcagttgggctaatctccccttcccttcctgatgtccatccgtctcacacgttggtgtctgggcgggctgagtcttctaggttgaagaggacaaaggtcagctggctcccccagcccgtgaacacctcagccaccaggaagactagaaaggctaacagtccaggagatgaatgccgctttgctccaacccttctttttcctctgaattccactgaccgcacgctccacttcacagtattaactggcatcaagcctcgactctcccaccccttgatctgctcacccacttcccttggaaacatccaaaacatcatgaagaggccctaagcacagagacatgggggcccacgtccagacgggccagtcagaacccagtgagcagaagcaaattgccctgcggttcaccaggctccagttaaacactcctccgtgacctgacatttcaaatcttcccctcttcctctgaacaatgtctcttcaaatgggaaggagggagcccacaaaagactagaggatgctctagatgattcgtgggctaagtaaggactaggttggcatccctctgcttgagagcttggtcctagtgacagcagcctatttgctaaggtgactcaatggcagattcggccaggtatgcaattgggcatccagggagctggcctctcctgcagggagcttctcttggggcttctgatgtggcagctccatgcatgggggtagaggaggccattgggtgaggactaggagaatgtgcactaatgtttgctgagcgtctgtggggctggcatcgcccaatacttcccttcccttcccttcggtgaagctggctatttcacccctttcttcaactggggcctagcactttgtgggtctggggacagcgtgtgagcacccagcgcacacagcacagtgcactgaagatgtggccggagcccagtggggatgctttcagagggggtgcagcctgtgatgcctgagcagccgcccagctttgttcagggtttctctggcctcctgctgtccctccacccacttccagctggctagaattgggtgctgggggcatgcatcacagggggagggggcaggctgaggaactgggtggtgtggtgaaatttcctggggaaggtaccacctgccagtcactcttacgccacctcactgtgcccagcagcttctgggagggggcaaatgtccctgcattgaagaacctaagccacgccccaggtgcgccgatggcaaaaggatggattgtggggaagcggatggggtcacctctgggagggaattttcttgcttaaataccagaggcaagccaaagatttagttaacagatttcagaagcacaggagagctctgaggatgtgggagagaagctggctaagggctggacagtcagtgactcgacattccccgagcccatgagatgccacctgacgtcgcatcccaggcctctgggatctagaaaatgacaaccttgatggtgaccatgttgtcagaagcccaatcaaggctttgattcttctttaaacttttgttctgtggtggatctttcttgacgtctcttgttgggatagagatgacagaaacaattttcctacttcctaagtctttcctttttttttttgcctgacaaaactggacatctggatgtccctccagtctacttatatactcacagagagaataagtttaaatattaaagagaaaacacaaagatacttggaataaatgtgcatttaaaaccctgactaaaatatcaacataatgatcataattacaatggtaataaaaataattagtacaataatattatctttatgagcagcatggaaatttcattcctgatctggaagaataaaaggaaagaaaatgtcaggtgaaagagtaagtagcctccaacttaagcagacagaataattttctttaaaatgaaaagaacattttaagctgtctttccccctaaaagatcagatctagaaagggctggaaatgaactgtgcccaggaatctgggggtgctctccagtaaggcgaactgaggctcatttgcagccaagacttggaactcgggatgagacctaatgggctattgctgccatctggctgccaaaaagtccctaatagatggattttccaggctgacccagctgtggggcgggggggggtcctctggcttctgtgtcctctgaagcgtttgctgccctcaccctctctgaactgaccattgtcctgctgtctcagagggctgcgcttccccacctccagataaagacagtattgataatggcccgagggaagggaatctccttgctgcaggcctcttgccggcacagcctccagcaggcacttggcaagactgcccggctgtgcccagcatggagcagtcatggtgtccttccttctcgctgaggcctggactaagctgtttccagtttggggacctgtttctttataagtaagaatttatggttggggtggggaagtttccagagttatttcacagctaagagctaagtaacgacttcgttactgagttaggttggatatcactacaaacacacctttcacagtagatccttgagggagactgcacagtgaggaagtaaagggagggaggatgaggatggggccgctgactcgggaaagatctctttgcaccttggaaacctgcctgtggggtcagctaaagactcaacatcagaagcaaacaattagaaccacccttttcggccccatccttggccagattctcctgccattcacattcacatatttcagagttatttactatgaagagagggaactccccacttctccacacctccatccccagaagtgtccaaagcctgagaaaacttccagaatgtatcaaaggtgcaaagagggcaaagggcagatttctttggaaattcaactgtgtgagtttttccaaagtgcagcgtcagacccccggccaccctcataagtgtccctccaaccttctgcccactagaaccctcagaaaccaaaaccaaaatcatgtcttgagcagacctgggtaatgtgaggagagaattcaacagcaaacagaggttggtggttgtctacagagggagggatctggcaagatcgttagagcaaaacagcccagggagccggaggagagagtggagccccgggcgaggctgagagctccaggctctcgtggaggcgggagggactgggggatgccgcctggggcgggagacggctgcctggcgaggccaacagtccggaaacctctggcctcacaaatggcggaactggggacagagtggggcaggggtgaagggtggggagtctctctgggcctccgcccacaaattacaactcaactactgccacaactcaactcccgccgtccccatctccagacgcacccgccgggcatctgtctcccatatttctttcgagatccacggactctctcctagctcctgctggcttccctggcatccttccgctagcaaacagcccaggaaagacaacgggcattaacattttaaaaagaaaaagaaaaagaaaaaaaaaaggccagcgtaaactgttacaacagcacaacagaagagctgagattgtgtctgactagcctcagtttcttggagtaccagtggaagtaaaccctcacgccgcgtctgtcgctcggtaaggcactaggagggaaggatgcagtgtcaagactgcgccagctagggtggcggcgccgagggccacgcggggagggcggcgcgtgcacacccacacgtgctcgctcacccgcacacctgcaccgccacattggttacatgcctatgttatatcgcttttttttgtgcaattacattgaggaatattctattggtatcattggagttgaacacaaggtaggagacaagggtgctgagtgctacattctactagggtgtctgtgacgaccgctagccctacgctacgcgactaggggtggattcaaagagaaaatacattttcagaaaagaaaaaaacctaaagtttgcaacacacattattaatgacatttgagaaacaacgttgcttagggatttatccagagtgctcagaaaaagaaaactcgccccgcgcccccgggggccttccagcagcctggccgtcccccgtctttcctgactagggagcccggactgggcttcgccaatcccacaccagctccaaacatcagcctcctcaggctgcagcccgacattctggagggctgttgaccctttcgagttctggaaaaatccctaaatcttatgttcaattaattaaaaatctatttgatttccatatcaggtgtccctgacagcagtcttccgtatcacttgctgccatatgaaaataatctttgaaaagttcataaagttcttcaaaaactggggccccccgtttctggaatcttcctgttgctctcttctcctttccagtttggcgtagaatgggttcttgagctgggttttttgttattgactttttttttttcctttttcttttttaaaataaaaaccatagatttcccaccctctttaatcccttccttttaaaaatgttctcttctctgctctacgtcctcccacttcccggttcaagtttcactggtgtcccgacccgtccccctgccctctgcccccccccccccccccgcccctgccccgtttgcattgtttgtgtgcggcatcttcagtataaaaggccagcgcccacggtcccaggagcgcctccctccttctctccctcctccctcgggccattctctccctccctccctccctccctcccctccagtgtttatatgtaagggtactggttgaccttggcggggctcagtgggtatccagtgtagacggtggaggctggcgaggcgctgatgtaggtctggtgggcaaattgggctggatactgactcgggtggatggtgggcgagggcaggacccgggggcccatgctcacggggacctggtggacgatgctggctgggtaggcagtgtgctgcacggtgtggcgcgcagagccttgcgaggccaccaggtgggccacggtgccggtggagcccagggccgccggcgcagtgtaggtgtagaggtggggctgggtggggaggtgggcagcggcagcggctgcagccagatgcgggtgcacagtgccgtggctggggctgttgtgcgggaaggagtacggagcctgggccatggtgggagtgatgtaggcctgctgccttcggtggctcccagtgcggtccgtggtgatgtgctgctgagcctggctgagattgagtggctgctgctgctggaagtgggggcccggccgctgctgccggtaggtgatggctccagatgagctccctgaagagtgaccgctggtggaggtcacgttgctggaggacttggacttgtaggaggacgagtggtgactggtgttgactggcaccaggctatcacactccaccaatacttcgctggcctgggttttcaggggtggcacgatgatggttcgggggttccccgtgcagtgattctccaggctccccttggtgtcaaaggcattggcattgttgtgcccagcacgctgctgcacggagtaggggctggtgttgctggaggagtcggagtagggggagtcgtggactgtgacacagctgatgacgttttttctttgcttggagacagtgctggtgggggcgtgtttctgttcctcctcctcgtccgtgtcactgctgatggtgatgacgctgaccgtggggctgggagtgtcgggaatgacaattgtctgccgctgccgttcccgggtggtgctggaggccacgtcgccccacccacaggtgaccgaggtgctgcaggccgggctactgtgcaccatggcacagcggggaggtgtgttctccttgacacgcttggatcgctgtggggagctgatggcctgagaggaggacacctcacaggtggagacatttctcacagatgactggtgctgcttactcttccgggaggaggtggtgctggttggctgctgccgcatcacgtgggccacacccacatttaagggctgtgctgctggaagggtcacatgaccggtcaatagtgcaggctgctgcatgatgggattataatggcttccgtgagcatgcgtatttctccagtccgccagctgctgggtgcctgccatggtctcgggaatcacggtggcatgctgcactgatgtgtgggtggccactccagtcagttgctgccatgctgggggaagcaggatctgctgggtcccacttggccaagcctgctgggcaagcagacctggttggatctgaagaggctgagctcctggggcttgagtgacgatgggaactgcattttccattcgcaccgagtagccagcgtgcttagagggagaggcctgcaagccttggaagccggggggacacacgatgagagcttgctggaacgggtcaggccgggcacaaatctgggctgttcctgtctgcaggggcatgctccgctgggccactgcagccatggatgccgctgagggctggttgtggacagtggtcagctggttgttaaaggtcatggtcaggttggtggacgtgctgggggccacgtgcgtgatgaaaggggttttgctctggttcaccgtgtcatacatattcacccgacgcttgcagatctccatgttctggaaacatgatttgacgtgtgtgctgtggggaaaatcgagtaagtgtgtcatggtgacaaagggatggttcagggtttcgattggagtgattctcttgtcagcatcaatggtcagcatcttcttcaacaggtcaatgaactcccgccggtcagccttttctaccaacatgtcgctcccttccaaatctgtcgtcatgttcacctgggccatatcatctaaacagttgaaaatgtactttcttgcttcttttgacttaatccctgtctctgcttcatggtcatctggtgtcttcagtctccacaaaggatatggtgagtccgtgtcacggttgaaaaacctagttgtctttgtcccggcgcttaataaatattcagcaggcaaaccctgtgtttgtgaaatataccgaatctgatcatactccgaagctcctggatataacggccaacccaggaacaattctgcaataacacagcccagggaccacatgtcaattgcctcacaaaatggtaaaccaaggatgatctcaggggccctgtaatatctggactgcaagtaggtggagcacacagccttggagacgtggctggctgaaccaaagtcgatgaccttgactctgtatggttgtctagatggatccaccagcatgatgttttctggtttgaggtcagcgtggataagacctaggcttttgagtttcatcagggctgtggctacctgctggagaactgggcgaatgtatttgaggggcaaggggctaaacttgttttgcttcagaaagtcatagaggttctgctccaacatctcgaagaccaagcacgtgtggttcttgtgctggaagcattcgtaggcccggacgaagttatagtcatcggcactctccgtgctcaaccgggccaggatgctcacttcaatctgaccttgtcgggcataggatgggtggttcttcaggatcttgatggctacgatctcattggtgccccgtttccagcacttgaccacttgcccaaacgtccctcggcccaagaactctaagacctcgtaggtgttggtcatggagcacagcacctcatgctgcaccagctgatagtcgccctcgctgttggagccgctgtttttggaggtggcagtagacgtggtggcagtggcgacagtggccccgcttgcattattctgaatcatgggtggatgctcctcgatgatctgcacgctgcttgtgttctcgatctcctcgctcttacgcttgagtccacatttttggtaggtatcaaggaggctcacagtgcttcgacgcattaggttgtgtggtccgccgaggacttgcccggtgacagaagtgctgcttgctgaggtgaccacgatgtgcccggtgcttcctgggaagacgatggtctgctcgtaaggtaggcttgggtttgggaccggcaaggaggtgctgacggttgtggtggctggctgcgacagggggatgttcttgctctggctatacactttgctgtgggagccgtacccagtcatgtcccagttggaactcggctctattttcagtttcttcacactacagaaggcacttgattgaagggtgtgaggggagaaaacttgcacatgtgaggccatacctgggagtggaactgccaggtcaggtggcgactctatgtttaaccttttgaggacctgacacttgttttccaaagtggcctcctgaagtccccaggagtcatgcaaagtcccccagaggtcccaggcaaagcgcacagaaggcccttctgcagagatgctgcccttctgtccttcggtaaaataccagcctaaattcaaagcaggagtcagggtttgtttgatttgaggtaaataaattagagaagctgtgactcgctcagtgccagcagcatgcttagcctggtatcgccccggagaaagagccagcacctggcatggcagacgagggttggcacaatgcatgcttgcttgccagatgaagaggcgctctgtgcaaagtgcagctgcagcaggacgcaaactggtgctctctctaccgtccctcaccagggcaaagctgtctgtgctcctggtcaaagcctcggaggacttatttgctgtcatccacacactgtgctccggaaagtgcctgctcagaaactggcagggagaagacccggagggagtgaggaccatgagaaatcagagagcaactagacaaggaagatatcaaaagagacgggtccttcgaggcctgcacacctgttagtcctaatatatttcagagcaagggatcagactggtgcacacatgggctgaagcccagggaaggagccaagtccaccaccaatgcaactggtgagtcagtatcaggcatgtgtcccctccaagctggcagtaaacaaacactcacacttcatgtttgggcactggactaaattaccaggcaaaagtacaaattccggccaggcgcggtggctcatgcctataatcccagcactttgaga

SEQ ID NO: 16235 - RNA, 13704 nt, Homo sapiens
  source 1..13704: mol_type = other RNA
ggaggccggggtggggcggggcgggggtgtgctctctgttccatttgttagttacaggaagctaccaaggatgcacatggtcaagtcactttctacttcccaagttcctccttataacctgagccaaacaatttcaacaatgacaatccattgccccttcagcccagcaggcgactctgacagggaggtgtgaccaccagtctcaaggctgagtggggccttcttgctggctctcgcgctttctgggagtcctgggtgccttggcccagggcagtggtgacagcagggtggaggcagaggtggccccggggacagtgaccctatataaggaagggggcggtgccaggagagattcgtttggagattggttacaaggaagcgagggagagcagaggcagagccctttttcagatacaacatacttacttttcaaatgaacaaaaggcaatttctatgttttaaaaatataagccccaaaaacaatgacacaaaattcatttggttaattcatgtaaaggaaaaaacagcaacaccaccacacaaacaggaaagtgggagtatgattaggaggggtgagatgaaaactattttacagtaacatttccaccaaaagactgtcctaagaacacgctgtcaatacagttcacagggaaaaagcaaatgtggtatttttttgtattttttaaaagctccctggtcccaggtgttttgcagttttcaaggtcttatctgctaaaggaatgccctttaggtcacagcaggtcctctgcagtttggtggtggcacaagagaaaacataaaagaaaccaagactcagggaaactgccattcccccagtctgtttctgcatgacagtggggcccattcctgtctcgaagcatcttcttgttccaaatatgatgtctgtttagagtgggtctcaatggaccaggctgagctgcccctctgtctctgcctcctcctgctcagccctgaccatctctgagaggatgctaaggtccccctcccaccgaactagactttgagtctaagctggacaatgagtaaaacgtaaacatagccttttacattgattttgcttttaaggggaaaacgaataaatgacagcagatatatggaaaacccagccagcgaccatgggaataggggtatatggtcctcccctacaaaacgctgatcaaaatatcacccccggcccagaagtagcagctgtgccttcatggtcacctgaatcccagtctcttctactgcctggtgcctggaaatcagtggatctattaataagttaaatattcaaatcaagacaaaaatcaatgaaccaggttatctgttctcaatgactcttccaagatgtcagagagaaggccttgaagacaagtgtttagacgacacgcatgagaccttcgcatctggcccgggctgcggactcacaccttttccctccatctggattgcctttcatgttctcttgagttcacgtggaaagtaataatccagagggaagtgcgcatgctggactacagaagagtctgggacaacacacttgccttgggggagacacaacctccaactaagaggcattcactggggtttgcggatgtcagttataaacagaacttttctttaaaaagtaccagtctaaatgtaaactataaaacactttaactataaaacgtagccagaaatatgcttaagtatccacagtcaattgtttagtttactcatttaaaatgtgactgttttgatagcttagaaggctaacagcattttacagtagctaaaaacatatatacttaacatgtgcatttgaacatcgcatttgagtacaacacacaaagaataatctcttccttggtttaatttttgttgtaaagatgagctattttcagaattcacttaagcaacgatgaccgggggtatgaagtaatcattattttcagcccacagagaattcatagtctttaaattccaagatcaagctggctacatgatttcaaaaaaggctaaaaccaggatgaatgcccacatttgaggtaattattgccattaggtcacagtttgtgtaagataatgtatctaaaaccttctaaaaaaaaaaaaaatctttaggtgttctgccagaattccagaatacctattgaaaccaaccaggatctcaaactccgattagttaggtttgcttccaatggagttaaagttctaaaagattctagaacttgtgtaaactacctaagaatttaggcaaacaagcctggagccagtcaacaaagaaggttttaaatgaaaaaaggaacaagaaacccactcaaaacaactgaacaaatatttcataataaatgataatagttattttaaaaaattaaaaatctagtcctaagcatttctacattctcaccatctttcaatcaaaataaaaatgcatctgtatttctgttaatctcataccagggcaagagacacgccttccttttatcatgaaagctggctggttttcctgtttatacaattgttgctatttctttgagaagagtatctcaaaagaaaacattcttttgttcctctaagtcttgtctttcttccacctctacttctttttttttttcttttttttttcttttttttaacagaaagaaaaaagttcctggacaccagacccacatatggtatttacaaatttggtgtgaaccctgcctctggttctgcccagagctgaagagtgaatctattacagagatcagagctgtcaggataattatcaagtgcagtaaaaaatagcattttgaaaaaaatatatacctttagtattgcctttctagaattaactataagcaagaaaaacttattttttaaagaagaaaagaatactttttcactcttacttataagagctggttgtagcagcactactaaagctagttggtatgctggaaagaaatctaaaaggaattctatgaatcaaaagaaactctccagagattttctctaaaaatcaaacgaattctgccccttttgcctaaatccaactcaggagccccctctttgcacagtcctttagctgagtcccacggtgcatgggatggcacagggtgatgctgtgtaaaggcctttctttgctcagacatgcaggagacagctgtggctaatggctgcaagctcagttctggagctgggcagactcaggttcaagccctcctcgcccctcaagagttgtgtggctctgggcagtttccttggctgtagggggactaatattgccgatctcacagggctacggagaagatgaaacaggacaacccatgagcaattcccagcacagtgtgtggcatgcaggaagcgggagtatcactaaatggttcatagaaatatgaggccacgcattgctattaattaaaaaaagttaaaagattaaaaatcacatctcaggaagggcctgatgaacaaaaaagggaaccttggggattctggcccatcactgctttatccttccttcaacacctgccacttctcagagcatccggtcagctcccttatctataaatgggggctgttatccccctccctgtgggatggctgttggggccccttgagacaacgctcataaaggccttagcccgggagtcatgaaagcattcaacaaatgttggctattatttacttgagagatattgcaaattttaacaaataagggacagtcagtgtcatgttcaacacagggatctgagatgaggggctcccagaggcttgggcaagtccagcggggggcatcgggaagaccctctctggtgctggtgttctgggacgggagccctgcagggggcacttctctgcaaactctcactgggtttgagggaagaacggcctggagttcttttttgaacttttcagaagctgcaacaagagaaacctctactatgctgggtccctctagtgagccacggtgccaaaagcctccaataggttttttttgcatttaaatcctgtttcaccgccttccattctctagtggcctgagattttactgagtctggtctgtggagatgagaagtgagagttctaaggcatcaaagtggaaaagtactgctattccgagcccagcccccgcgtgctctacgcccttgatgcaactgaactcctggcagccctgctttgctctctcccatggtggcctgggattagtcaagcccacgtattggtatggcaccttgtctcccgatagcagcagcatcgaaggggtcacctccactcctcttaaaagaatagcacagttttgaaataaatgcattttttttttttaaaaaaaaggacagagaggaaagagaaagacaaatagaattgcatcactaatgatgtcattattgcctggaaaggaacgaagggaaggccattttgtccatttctggaggcgtctttgagaagggttctttggctaaagaaaggaacagtttcaccttcctttccaatttggtaaggacatctctggcctgctcaagtttgaagcttccccatcagaagtctgtaaaacacaccagaaggaaaagacacagacagggaatgaagcctgcaaagtccctggggctggaatgtcttgtggccaagtcactcctgctggcgctgtggagtcccaggctggcctgcagaaggaacccttacctctcctcaattctctctgctagttgagagcaccgagccatttccttctttccattttctgtcctagggtctacttgacaggccaacaagagtggtggtcccacaccccaccctgccctcagcatcagacaaagagaacctgggacaaaagctggggcgagctgggtccccacgtcgctctctcaaccatgagccatcagtaatacttcccgaagcctcctcatctcctccctccagtttccaagaaagtttgttccactcactcacacatgctcacacggcctaaatcttccaccccaagcttgttccaatatgagtgtttgccattcccaaggtccaaccaagggaaatcgttctgtcagcagttgggctaatctccccttcccttcctgatgtccatccgtctcacacgttggtgtctgggcgggctgagtcttctaggttgaagaggacaaaggtcagctggctcccccagcccgtgaacacctcagccaccaggaagactagaaaggctaacagtccaggagatgaatgccgctttgctccaacccttctttttcctctgaattccactgaccgcacgctccacttcacagtattaactggcatcaagcctcgactctcccaccccttgatctgctcacccacttcccttggaaacatccaaaacatcatgaagaggccctaagcacagagacatgggggcccacgtccagacgggccagtcagaacccagtgagcagaagcaaattgccctgcggttcaccaggctccagttaaacactcctccgtgacctgacatttcaaatcttcccctcttcctctgaacaatgtctcttcaaatgggaaggagggagcccacaaaagactagaggatgctctagatgattcgtgggctaagtaaggactaggttggcatccctctgcttgagagcttggtcctagtgacagcagcctatttgctaaggtgactcaatggcagattcggccaggtatgcaattgggcatccagggagctggcctctcctgcagggagcttctcttggggcttctgatgtggcagctccatgcatgggggtagaggaggccattgggtgaggactaggagaatgtgcactaatgtttgctgagcgtctgtggggctggcatcgcccaatacttcccttcccttcccttcggtgaagctggctatttcacccctttcttcaactggggcctagcactttgtgggtctggggacagcgtgtgagcacccagcgcacacagcacagtgcactgaagatgtggccggagcccagtggggatgctttcagagggggtgcagcctgtgatgcctgagcagccgcccagctttgttcagggtttctctggcctcctgctgtccctccacccacttccagctggctagaattgggtgctgggggcatgcatcacagggggagggggcaggctgaggaactgggtggtgtggtgaaatttcctggggaaggtaccacctgccagtcactcttacgccacctcactgtgcccagcagcttctgggagggggcaaatgtccctgcattgaagaacctaagccacgccccaggtgcgccgatggcaaaaggatggattgtggggaagcggatggggtcacctctgggagggaattttcttgcttaaataccagaggcaagccaaagatttagttaacagatttcagaagcacaggagagctctgaggatgtgggagagaagctggctaagggctggacagtcagtgactcgacattccccgagcccatgagatgccacctgacgtcgcatcccaggcctctgggatctagaaaatgacaaccttgatggtgaccatgttgtcagaagcccaatcaaggctttgattcttctttaaacttttgttctgtggtggatctttcttgacgtctcttgttgggatagagatgacagaaacaattttcctacttcctaagtctttcctttttttttttgcctgacaaaactggacatctggatgtccctccagtctacttatatactcacagagagaataagtttaaatattaaagagaaaacacaaagatacttggaataaatgtgcatttaaaaccctgactaaaatatcaacataatgatcataattacaatggtaataaaaataattagtacaataatattatctttatgagcagcatggaaatttcattcctgatctggaagaataaaaggaaagaaaatgtcaggtgaaagagtaagtagcctccaacttaagcagacagaataattttctttaaaatgaaaagaacattttaagctgtctttccccctaaaagatcagatctagaaagggctggaaatgaactgtgcccaggaatctgggggtgctctccagtaaggcgaactgaggctcatttgcagccaagacttggaactcgggatgagacctaatgggctattgctgccatctggctgccaaaaagtccctaatagatggattttccaggctgacccagctgtggggcgggggggggtcctctggcttctgtgtcctctgaagcgtttgctgccctcaccctctctgaactgaccattgtcctgctgtctcagagggctgcgcttccccacctccagataaagacagtattgataatggcccgagggaagggaatctccttgctgcaggcctcttgccggcacagcctccagcaggcacttggcaagactgcccggctgtgcccagcatggagcagtcatggtgtccttccttctcgctgaggcctggactaagctgtttccagtttggggacctgtttctttataagtaagaatttatggttggggtggggaagtttccagagttatttcacagctaagagctaagtaacgacttcgttactgagttaggttggatatcactacaaacacacctttcacagtagatccttgagggagactgcacagtgaggaagtaaagggagggaggatgaggatggggccgctgactcgggaaagatctctttgcaccttggaaacctgcctgtggggtcagctaaagactcaacatcagaagcaaacaattagaaccacccttttcggccccatccttggccagattctcctgccattcacattcacatatttcagagttatttactatgaagagagggaactccccacttctccacacctccatccccagaagtgtccaaagcctgagaaaacttccagaatgtatcaaaggtgcaaagagggcaaagggcagatttctttggaaattcaactgtgtgagtttttccaaagtgcagcgtcagacccccggccaccctcataagtgtccctccaaccttctgcccactagaaccctcagaaaccaaaaccaaaatcatgtcttgagcagacctgggtaatgtgaggagagaattcaacagcaaacagaggttggtggttgtctacagagggagggatctggcaagatcgttagagcaaaacagcccagggagccggaggagagagtggagccccgggcgaggctgagagctccaggctctcgtggaggcgggagggactgggggatgccgcctggggcgggagacggctgcctggcgaggccaacagtccggaaacctctggcctcacaaatggcggaactggggacagagtggggcaggggtgaagggtggggagtctctctgggcctccgcccacaaattacaactcaactactgccacaactcaactcccgccgtccccatctccagacgcacccgccgggcatctgtctcccatatttctttcgagatccacggactctctcctagctcctgctggcttccctggcatccttccgctagcaaacagcccaggaaagacaacgggcattaacattttaaaaagaaaaagaaaaagaaaaaaaaaaggccagcgtaaactgttacaacagcacaacagaagagctgagattgtgtctgactagcctcagtttcttggagtaccagtggaagtaaaccctcacgccgcgtctgtcgctcggtaaggcactaggagggaaggatgcagtgtcaagactgcgccagctagggtggcggcgccgagggccacgcggggagggcggcgcgtgcacacccacacgtgctcgctcacccgcacacctgcaccgccacattggttacatgcctatgttatatcgcttttttttgtgcaattacattgaggaatattctattggtatcattggagttgaacacaaggtaggagacaagggtgctgagtgctacattctactagggtgtctgtgacgaccgctagccctacgctacgcgactaggggtggattcaaagagaaaatacattttcagaaaagaaaaaaacctaaagtttgcaacacacattattaatgacatttgagaaacaacgttgcttagggatttatccagagtgctcagaaaaagaaaactcgccccgcgcccccgggggccttccagcagcctggccgtcccccgtctttcctgactagggagcccggactgggcttcgccaatcccacaccagctccaaacatcagcctcctcaggctgcagcccgacattctggagggctgttgaccctttcgagttctggaaaaatccctaaatcttatgttcaattaattaaaaatctatttgatttccatatcaggtgtccctgacagcagtcttccgtatcacttgctgccatatgaaaataatctttgaaaagttcataaagttcttcaaaaactggggccccccgtttctggaatcttcctgttgctctcttctcctttccagtttggcgtagaatgggttcttgagctgggttttttgttattgactttttttttttcctttttcttttttaaaataaaaaccatagatttcccaccctctttaatcccttccttttaaaaatgttctcttctctgctctacgtcctcccacttcccggttcaagtttcactggtgtcccgacccgtccccctgccctctgcccccccccccccccccgcccctgccccgtttgcattgtttgtgtgcggcatcttcagtataaaaggccagcgcccacggtcccaggagcgcctccctccttctctccctcctccctcgggccattctctccctccctccctccctccctcccctccagtgtttatatgtaagggtactggttgaccttggcggggctcagtgggtatccagtgtagacggtggaggctggcgaggcgctgatgtaggtctggtgggcaaattgggctggatactgactcgggtggatggtgggcgagggcaggacccgggggcccatgctcacggggacctggtggacgatgctggctgggtaggcagtgtgctgcacggtgtggcgcgcagagccttgcgaggccaccaggtgggccacggtgccggtggagcccagggccgccggcgcagtgtaggtgtagaggtggggctgggtggggaggtgggcagcggcagcggctgcagccagatgcgggtgcacagtgccgtggctggggctgttgtgcgggaaggagtacggagcctgggccatggtgggagtgatgtaggcctgctgccttcggtggctcccagtgcggtccgtggtgatgtgctgctgagcctggctgagattgagtggctgctgctgctggaagtgggggcccggccgctgctgccggtaggtgatggctccagatgagctccctgaagagtgaccgctggtggaggtcacgttgctggaggacttggacttgtaggaggacgagtggtgactggtgttgactggcaccaggctatcacactccaccaatacttcgctggcctgggttttcaggggtggcacgatgatggttcgggggttccccgtgcagtgattctccaggctccccttggtgtcaaaggcattggcattgttgtgcccagcacgctgctgcacggagtaggggctggtgttgctggaggagtcggagtagggggagtcgtggactgtgacacagctgatgacgttttttctttgcttggagacagtgctggtgggggcgtgtttctgttcctcctcctcgtccgtgtcactgctgatggtgatgacgctgaccgtggggctgggagtgtcgggaatgacaattgtctgccgctgccgttcccgggtggtgctggaggccacgtcgccccacccacaggtgaccgaggtgctgcaggccgggctactgtgcaccatggcacagcggggaggtgtgttctccttgacacgcttggatcgctgtggggagctgatggcctgagaggaggacacctcacaggtggagacatttctcacagatgactggtgctgcttactcttccgggaggaggtggtgctggttggctgctgccgcatcacgtgggccacacccacatttaagggctgtgctgctggaagggtcacatgaccggtcaatagtgcaggctgctgcatgatgggattataatggcttccgtgagcatgcgtatttctccagtccgccagctgctgggtgcctgccatggtctcgggaatcacggtggcatgctgcactgatgtgtgggtggccactccagtcagttgctgccatgctgggggaagcaggatctgctgggtcccacttggccaagcctgctgggcaagcagacctggttggatctgaagaggctgagctcctggggcttgagtgacgatgggaactgcattttccattcgcaccgagtagccagcgtgcttagagggagaggcctgcaagccttggaagccggggggacacacgatgagagcttgctggaacgggtcaggccgggcacaaatctgggctgttcctgtctgcaggggcatgctccgctgggccactgcagccatggatgccgctgagggctggttgtggacagtggtcagctggttgttaaaggtcatggtcaggttggtggacgtgctgggggccacgtgcgtgatgaaaggggttttgctctggttcaccgtgtcatacatattcacccgacgcttgcagatctccatgttctggaaacatgatttgacgtgtgtgctgtggggaaaatcgagtaagtgtgtcatggtgacaaagggatggttcagggtttcgattggagtgattctcttgtcagcatcaatggtcagcatcttcttcaacaggtcaatgaactcccgccggtcagccttttctaccaacatgtcgctcccttccaaatctgtcgtcatgttcacctgggccatatcatctaaacagttgaaaatgtactttcttgcttcttttgacttaatccctgtctctgcttcatggtcatctggtgtcttcagtctccacaaaggatatggtgagtccgtgtcacggttgaaaaacctagttgtctttgtcccggcgcttaataaatattcagcaggcaaaccctgtgtttgtgaaatataccgaatctgatcatactccgaagctcctggatataacggccaacccaggaacaattctgcaataacacagcccagggaccacatgtcaattgcctcacaaaatggtaaaccaaggatgatctcaggggccctgtaatatctggactgcaagtaggtggagcacacagccttggagacgtggctggctgaaccaaagtcgatgaccttgactctgtatggttgtctagatggatccaccagcatgatgttttctggtttgaggtcagcgtggataagacctaggcttttgagtttcatcagggctgtggctacctgctggagaactgggcgaatgtatttgaggggcaaggggctaaacttgttttgcttcagaaagtcatagaggttctgctccaacatctcgaagaccaagcacgtgtggttcttgtgctggaagcattcgtaggcccggacgaagttatagtcatcggcactctccgtgctcaaccgggccaggatgctcacttcaatctgaccttgtcgggcataggatgggtggttcttcaggatcttgatggctacgatctcattggtgccccgtttccagcacttgaccacttgcccaaacgtccctcggcccaagaactctaagacctcgtaggtgttggtcatggagcacagcacctcatgctgcaccagctgatagtcgccctcgctgttggagccgctgtttttggaggtggcagtagacgtggtggcagtggcgacagtggccccgcttgcattattctgaatcatgggtggatgctcctcgatgatctgcacgctgcttgtgttctcgatctcctcgctcttacgcttgagtccacatttttggtaggtatcaaggaggctcacagtgcttcgacgcattaggttgtgtggtccgccgaggacttgcccggtgacagaagtgctgcttgctgaggtgaccacgatgtgcccggtgcttcctgggaagacgatggtctgctcgtaaggtaggcttgggtttgggaccggcaaggaggtgctgacggttgtggtggctggctgcgacagggggatgttcttgctctggctatacactttgctgtgggagccgtacccagtcatgtcccagttggaactcggctctattttcagtttcttcacactacagaaggcacttgattgaagggtgtgaggggagaaaacttgcacatgtgaggccataccttcgtacacgggggccatcggggccggggtgtccgcggttcatggcaacggggacgggaaagcggcgcgcgagctcggcccccccagcctcagtcggaatctgccatcttgagcctgtgtctccgctctcggcgcagccgaggccgcccgcgcccgcatcaccgcctcccgtggccggcgccgggggagggggccgggcgcgccgccgccgccgccgccgccgctgccgcccgggcccggcgcggggggctcggggctcggggctcggggcggccgggcgggcggagcggccgaggccgaggcgccgagcggccgcggcccccgagcggatccgcggaggggcgggagccgggggcagcgcgcggccagggccggcggggctcagctcagcat

SEQ ID NO: 16236 - RNA, 14255 nt, Homo sapiens
  source 1..14255: mol_type = other RNA
ggaggccggggtggggcggggcgggggtgtgctctctgttccatttgttagttacaggaagctaccaaggatgcacatggtcaagtcactttctacttcccaagttcctccttataacctgagccaaacaatttcaacaatgacaatccattgccccttcagcccagcaggcgactctgacagggaggtgtgaccaccagtctcaaggctgagtggggccttcttgctggctctcgcgctttctgggagtcctgggtgccttggcccagggcagtggtgacagcagggtggaggcagaggtggccccggggacagtgaccctatataaggaagggggcggtgccaggagagattcgtttggagattggttacaaggaagcgagggagagcagaggcagagccctttttcagatacaacatacttacttttcaaatgaacaaaaggcaatttctatgttttaaaaatataagccccaaaaacaatgacacaaaattcatttggttaattcatgtaaaggaaaaaacagcaacaccaccacacaaacaggaaagtgggagtatgattaggaggggtgagatgaaaactattttacagtaacatttccaccaaaagactgtcctaagaacacgctgtcaatacagttcacagggaaaaagcaaatgtggtatttttttgtattttttaaaagctccctggtcccaggtgttttgcagttttcaaggtcttatctgctaaaggaatgccctttaggtcacagcaggtcctctgcagtttggtggtggcacaagagaaaacataaaagaaaccaagactcagggaaactgccattcccccagtctgtttctgcatgacagtggggcccattcctgtctcgaagcatcttcttgttccaaatatgatgtctgtttagagtgggtctcaatggaccaggctgagctgcccctctgtctctgcctcctcctgctcagccctgaccatctctgagaggatgctaaggtccccctcccaccgaactagactttgagtctaagctggacaatgagtaaaacgtaaacatagccttttacattgattttgcttttaaggggaaaacgaataaatgacagcagatatatggaaaacccagccagcgaccatgggaataggggtatatggtcctcccctacaaaacgctgatcaaaatatcacccccggcccagaagtagcagctgtgccttcatggtcacctgaatcccagtctcttctactgcctggtgcctggaaatcagtggatctattaataagttaaatattcaaatcaagacaaaaatcaatgaaccaggttatctgttctcaatgactcttccaagatgtcagagagaaggccttgaagacaagtgtttagacgacacgcatgagaccttcgcatctggcccgggctgcggactcacaccttttccctccatctggattgcctttcatgttctcttgagttcacgtggaaagtaataatccagagggaagtgcgcatgctggactacagaagagtctgggacaacacacttgccttgggggagacacaacctccaactaagaggcattcactggggtttgcggatgtcagttataaacagaacttttctttaaaaagtaccagtctaaatgtaaactataaaacactttaactataaaacgtagccagaaatatgcttaagtatccacagtcaattgtttagtttactcatttaaaatgtgactgttttgatagcttagaaggctaacagcattttacagtagctaaaaacatatatacttaacatgtgcatttgaacatcgcatttgagtacaacacacaaagaataatctcttccttggtttaatttttgttgtaaagatgagctattttcagaattcacttaagcaacgatgaccgggggtatgaagtaatcattattttcagcccacagagaattcatagtctttaaattccaagatcaagctggctacatgatttcaaaaaaggctaaaaccaggatgaatgcccacatttgaggtaattattgccattaggtcacagtttgtgtaagataatgtatctaaaaccttctaaaaaaaaaaaaaatctttaggtgttctgccagaattccagaatacctattgaaaccaaccaggatctcaaactccgattagttaggtttgcttccaatggagttaaagttctaaaagattctagaacttgtgtaaactacctaagaatttaggcaaacaagcctggagccagtcaacaaagaaggttttaaatgaaaaaaggaacaagaaacccactcaaaacaactgaacaaatatttcataataaatgataatagttattttaaaaaattaaaaatctagtcctaagcatttctacattctcaccatctttcaatcaaaataaaaatgcatctgtatttctgttaatctcataccagggcaagagacacgccttccttttatcatgaaagctggctggttttcctgtttatacaattgttgctatttctttgagaagagtatctcaaaagaaaacattcttttgttcctctaagtcttgtctttcttccacctctacttctttttttttttcttttttttttcttttttttaacagaaagaaaaaagttcctggacaccagacccacatatggtatttacaaatttggtgtgaaccctgcctctggttctgcccagagctgaagagtgaatctattacagagatcagagctgtcaggataattatcaagtgcagtaaaaaatagcattttgaaaaaaatatatacctttagtattgcctttctagaattaactataagcaagaaaaacttattttttaaagaagaaaagaatactttttcactcttacttataagagctggttgtagcagcactactaaagctagttggtatgctggaaagaaatctaaaaggaattctatgaatcaaaagaaactctccagagattttctctaaaaatcaaacgaattctgccccttttgcctaaatccaactcaggagccccctctttgcacagtcctttagctgagtcccacggtgcatgggatggcacagggtgatgctgtgtaaaggcctttctttgctcagacatgcaggagacagctgtggctaatggctgcaagctcagttctggagctgggcagactcaggttcaagccctcctcgcccctcaagagttgtgtggctctgggcagtttccttggctgtagggggactaatattgccgatctcacagggctacggagaagatgaaacaggacaacccatgagcaattcccagcacagtgtgtggcatgcaggaagcgggagtatcactaaatggttcatagaaatatgaggccacgcattgctattaattaaaaaaagttaaaagattaaaaatcacatctcaggaagggcctgatgaacaaaaaagggaaccttggggattctggcccatcactgctttatccttccttcaacacctgccacttctcagagcatccggtcagctcccttatctataaatgggggctgttatccccctccctgtgggatggctgttggggccccttgagacaacgctcataaaggccttagcccgggagtcatgaaagcattcaacaaatgttggctattatttacttgagagatattgcaaattttaacaaataagggacagtcagtgtcatgttcaacacagggatctgagatgaggggctcccagaggcttgggcaagtccagcggggggcatcgggaagaccctctctggtgctggtgttctgggacgggagccctgcagggggcacttctctgcaaactctcactgggtttgagggaagaacggcctggagttcttttttgaacttttcagaagctgcaacaagagaaacctctactatgctgggtccctctagtgagccacggtgccaaaagcctccaataggttttttttgcatttaaatcctgtttcaccgccttccattctctagtggcctgagattttactgagtctggtctgtggagatgagaagtgagagttctaaggcatcaaagtggaaaagtactgctattccgagcccagcccccgcgtgctctacgcccttgatgcaactgaactcctggcagccctgctttgctctctcccatggtggcctgggattagtcaagcccacgtattggtatggcaccttgtctcccgatagcagcagcatcgaaggggtcacctccactcctcttaaaagaatagcacagttttgaaataaatgcattttttttttttaaaaaaaaggacagagaggaaagagaaagacaaatagaattgcatcactaatgatgtcattattgcctggaaaggaacgaagggaaggccattttgtccatttctggaggcgtctttgagaagggttctttggctaaagaaaggaacagtttcaccttcctttccaatttggtaaggacatctctggcctgctcaagtttgaagcttccccatcagaagtctgtaaaacacaccagaaggaaaagacacagacagggaatgaagcctgcaaagtccctggggctggaatgtcttgtggccaagtcactcctgctggcgctgtggagtcccaggctggcctgcagaaggaacccttacctctcctcaattctctctgctagttgagagcaccgagccatttccttctttccattttctgtcctagggtctacttgacaggccaacaagagtggtggtcccacaccccaccctgccctcagcatcagacaaagagaacctgggacaaaagctggggcgagctgggtccccacgtcgctctctcaaccatgagccatcagtaatacttcccgaagcctcctcatctcctccctccagtttccaagaaagtttgttccactcactcacacatgctcacacggcctaaatcttccaccccaagcttgttccaatatgagtgtttgccattcccaaggtccaaccaagggaaatcgttctgtcagcagttgggctaatctccccttcccttcctgatgtccatccgtctcacacgttggtgtctgggcgggctgagtcttctaggttgaagaggacaaaggtcagctggctcccccagcccgtgaacacctcagccaccaggaagactagaaaggctaacagtccaggagatgaatgccgctttgctccaacccttctttttcctctgaattccactgaccgcacgctccacttcacagtattaactggcatcaagcctcgactctcccaccccttgatctgctcacccacttcccttggaaacatccaaaacatcatgaagaggccctaagcacagagacatgggggcccacgtccagacgggccagtcagaacccagtgagcagaagcaaattgccctgcggttcaccaggctccagttaaacactcctccgtgacctgacatttcaaatcttcccctcttcctctgaacaatgtctcttcaaatgggaaggagggagcccacaaaagactagaggatgctctagatgattcgtgggctaagtaaggactaggttggcatccctctgcttgagagcttggtcctagtgacagcagcctatttgctaaggtgactcaatggcagattcggccaggtatgcaattgggcatccagggagctggcctctcctgcagggagcttctcttggggcttctgatgtggcagctccatgcatgggggtagaggaggccattgggtgaggactaggagaatgtgcactaatgtttgctgagcgtctgtggggctggcatcgcccaatacttcccttcccttcccttcggtgaagctggctatttcacccctttcttcaactggggcctagcactttgtgggtctggggacagcgtgtgagcacccagcgcacacagcacagtgcactgaagatgtggccggagcccagtggggatgctttcagagggggtgcagcctgtgatgcctgagcagccgcccagctttgttcagggtttctctggcctcctgctgtccctccacccacttccagctggctagaattgggtgctgggggcatgcatcacagggggagggggcaggctgaggaactgggtggtgtggtgaaatttcctggggaaggtaccacctgccagtcactcttacgccacctcactgtgcccagcagcttctgggagggggcaaatgtccctgcattgaagaacctaagccacgccccaggtgcgccgatggcaaaaggatggattgtggggaagcggatggggtcacctctgggagggaattttcttgcttaaataccagaggcaagccaaagatttagttaacagatttcagaagcacaggagagctctgaggatgtgggagagaagctggctaagggctggacagtcagtgactcgacattccccgagcccatgagatgccacctgacgtcgcatcccaggcctctgggatctagaaaatgacaaccttgatggtgaccatgttgtcagaagcccaatcaaggctttgattcttctttaaacttttgttctgtggtggatctttcttgacgtctcttgttgggatagagatgacagaaacaattttcctacttcctaagtctttcctttttttttttgcctgacaaaactggacatctggatgtccctccagtctacttatatactcacagagagaataagtttaaatattaaagagaaaacacaaagatacttggaataaatgtgcatttaaaaccctgactaaaatatcaacataatgatcataattacaatggtaataaaaataattagtacaataatattatctttatgagcagcatggaaatttcattcctgatctggaagaataaaaggaaagaaaatgtcaggtgaaagagtaagtagcctccaacttaagcagacagaataattttctttaaaatgaaaagaacattttaagctgtctttccccctaaaagatcagatctagaaagggctggaaatgaactgtgcccaggaatctgggggtgctctccagtaaggcgaactgaggctcatttgcagccaagacttggaactcgggatgagacctaatgggctattgctgccatctggctgccaaaaagtccctaatagatggattttccaggctgacccagctgtggggcgggggggggtcctctggcttctgtgtcctctgaagcgtttgctgccctcaccctctctgaactgaccattgtcctgctgtctcagagggctgcgcttccccacctccagataaagacagtattgataatggcccgagggaagggaatctccttgctgcaggcctcttgccggcacagcctccagcaggcacttggcaagactgcccggctgtgcccagcatggagcagtcatggtgtccttccttctcgctgaggcctggactaagctgtttccagtttggggacctgtttctttataagtaagaatttatggttggggtggggaagtttccagagttatttcacagctaagagctaagtaacgacttcgttactgagttaggttggatatcactacaaacacacctttcacagtagatccttgagggagactgcacagtgaggaagtaaagggagggaggatgaggatggggccgctgactcgggaaagatctctttgcaccttggaaacctgcctgtggggtcagctaaagactcaacatcagaagcaaacaattagaaccacccttttcggccccatccttggccagattctcctgccattcacattcacatatttcagagttatttactatgaagagagggaactccccacttctccacacctccatccccagaagtgtccaaagcctgagaaaacttccagaatgtatcaaaggtgcaaagagggcaaagggcagatttctttggaaattcaactgtgtgagtttttccaaagtgcagcgtcagacccccggccaccctcataagtgtccctccaaccttctgcccactagaaccctcagaaaccaaaaccaaaatcatgtcttgagcagacctgggtaatgtgaggagagaattcaacagcaaacagaggttggtggttgtctacagagggagggatctggcaagatcgttagagcaaaacagcccagggagccggaggagagagtggagccccgggcgaggctgagagctccaggctctcgtggaggcgggagggactgggggatgccgcctggggcgggagacggctgcctggcgaggccaacagtccggaaacctctggcctcacaaatggcggaactggggacagagtggggcaggggtgaagggtggggagtctctctgggcctccgcccacaaattacaactcaactactgccacaactcaactcccgccgtccccatctccagacgcacccgccgggcatctgtctcccatatttctttcgagatccacggactctctcctagctcctgctggcttccctggcatccttccgctagcaaacagcccaggaaagacaacgggcattaacattttaaaaagaaaaagaaaaagaaaaaaaaaaggccagcgtaaactgttacaacagcacaacagaagagctgagattgtgtctgactagcctcagtttcttggagtaccagtggaagtaaaccctcacgccgcgtctgtcgctcggtaaggcactaggagggaaggatgcagtgtcaagactgcgccagctagggtggcggcgccgagggccacgcggggagggcggcgcgtgcacacccacacgtgctcgctcacccgcacacctgcaccgccacattggttacatgcctatgttatatcgcttttttttgtgcaattacattgaggaatattctattggtatcattggagttgaacacaaggtaggagacaagggtgctgagtgctacattctactagggtgtctgtgacgaccgctagccctacgctacgcgactaggggtggattcaaagagaaaatacattttcagaaaagaaaaaaacctaaagtttgcaacacacattattaatgacatttgagaaacaacgttgcttagggatttatccagagtgctcagaaaaagaaaactcgccccgcgcccccgggggccttccagcagcctggccgtcccccgtctttcctgactagggagcccggactgggcttcgccaatcccacaccagctccaaacatcagcctcctcaggctgcagcccgacattctggagggctgttgaccctttcgagttctggaaaaatccctaaatcttatgttcaattaattaaaaatctatttgatttccatatcaggtgtccctgacagcagtcttccgtatcacttgctgccatatgaaaataatctttgaaaagttcataaagttcttcaaaaactggggccccccgtttctggaatcttcctgttgctctcttctcctttccagtttggcgtagaatgggttcttgagctgggttttttgttattgactttttttttttcctttttcttttttaaaataaaaaccatagatttcccaccctctttaatcccttccttttaaaaatgttctcttctctgctctacgtcctcccacttcccggttcaagtttcactggtgtcccgacccgtccccctgccctctgcccccccccccccccccgcccctgccccgtttgcattgtttgtgtgcggcatcttcagtataaaaggccagcgcccacggtcccaggagcgcctccctccttctctccctcctccctcgggccattctctccctccctccctccctccctcccctccagtgtttatatgtaagggtactggttgaccttggcggggctcagtgggtatccagtgtagacggtggaggctggcgaggcgctgatgtaggtctggtgggcaaattgggctggatactgactcgggtggatggtgggcgagggcaggacccgggggcccatgctcacggggacctggtggacgatgctggctgggtaggcagtgtgctgcacggtgtggcgcgcagagccttgcgaggccaccaggtgggccacggtgccggtggagcccagggccgccggcgcagtgtaggtgtagaggtggggctgggtggggaggtgggcagcggcagcggctgcagccagatgcgggtgcacagtgccgtggctggggctgttgtgcgggaaggagtacggagcctgggccatggtgggagtgatgtaggcctgctgccttcggtggctcccagtgcggtccgtggtgatgtgctgctgagcctggctgagattgagtggctgctgctgctggaagtgggggcccggccgctgctgccggtaggtgatggctccagatgagctccctgaagagtgaccgctggtggaggtcacgttgctggaggacttggacttgtaggaggacgagtggtgactggtgttgactggcaccaggctatcacactccaccaatacttcgctggcctgggttttcaggggtggcacgatgatggttcgggggttccccgtgcagtgattctccaggctccccttggtgtcaaaggcattggcattgttgtgcccagcacgctgctgcacggagtaggggctggtgttgctggaggagtcggagtagggggagtcgtggactgtgacacagctgatgacgttttttctttgcttggagacagtgctggtgggggcgtgtttctgttcctcctcctcgtccgtgtcactgctgatggtgatgacgctgaccgtggggctgggagtgtcgggaatgacaattgtctgccgctgccgttcccgggtggtgctggaggccacgtcgccccacccacaggtgaccgaggtgctgcaggccgggctactgtgcaccatggcacagcggggaggtgtgttctccttgacacgcttggatcgctgtggggagctgatggcctgagaggaggacacctcacaggtggagacatttctcacagatgactggtgctgcttactcttccgggaggaggtggtgctggttggctgctgccgcatcacgtgggccacacccacatttaagggctgtgctgctggaagggtcacatgaccggtcaatagtgcaggctgctgcatgatgggattataatggcttccgtgagcatgcgtatttctccagtccgccagctgctgggtgcctgccatggtctcgggaatcacggtggcatgctgcactgatgtgtgggtggccactccagtcagttgctgccatgctgggggaagcaggatctgctgggtcccacttggccaagcctgggcaagcagacctggttggatctgaagaggctgagctcctggggcttgagtgacgatgggaactgcattttccattcgcaccgagtagccagcgtgcttagagggagaggcctgcaagccttggaagccggggggacacacgatgagagcttgctggaacgggtcaggccgggcacaaatctgggctgttcctgtctgcaggggcatgctccgctgggccactgcagccatggatgccgctgagggctggtagagtgtagatgggtagtttagtatggagacttcgggattggctaaggaaatagtggcactggtagaggagggagcctggttgtggacagtggtcagctggttgttaaaggtcatggtcaggttggtggacgtgctgggggccacgtgcgtgatgaaaggggttttgctctggttcaccgtgtcatacatattcacccgacgcttgcagatctccatgttctggaaacatgatttgacgtgtgtgctgtggggaaaatcgagtaagtgtgtcatggtgacaaagggatggttcagggtttcgattggagtgattctcttgtcagcatcaatggtcagcatcttcttcaacaggtcaatgaactcccgccggtcagccttttctaccaacatgtcgctcccttccaaatctgtcgtcatgttcacctgggccatatcatctaaacagttgaaaatgtactttcttgcttcttttgacttaatccctgtctctgcttcatggtcatctggtgtcttcagtctccacaaaggatatggtgagtccgtgtcacggttgaaaaacctagttgtctttgtcccggcgcttaataaatattcagcaggcaaaccctgtgtttgtgaaatataccgaatctgatcatactccgaagctcctggatataacggccaacccaggaacaattctgcaataacacagcccagggaccacatgtcaattgcctcacaaaatggtaaaccaaggatgatctcaggggccctgtaatatctggactgcaagtaggtggagcacacagccttggagacgtggctggctgaaccaaagtcgatgaccttgactctgtatggttgtctagatggatccaccagcatgatgttttctggtttgaggtcagcgtggataagacctaggcttttgagtttcatcagggctgtggctacctgctggagaactgggcgaatgtatttgaggggcaaggggctaaacttgttttgcttcagaaagtcatagaggttctgctccaacatctcgaagaccaagcacgtgtggttcttgtgctggaagcattcgtaggcccggacgaagttatagtcatcggcactctccgtgctcaaccgggccaggatgctcacttcaatctgaccttgtcgggcataggatgggtggttcttcaggatcttgatggctacgatctcattggtgccccgtttccagcacttgaccacttgcccaaacgtccctcggcccaagaactctaagacctcgtaggtgttggtcatggagcacagcacctcatgctgcaccagctgatagtcgccctcgctgttggagccgctgtttttggaggtggcagtagacgtggtggcagtggcgacagtggccccgcttgcattattctgaatcatgggtggatgctcctcgatgatctgcacgctgcttgtgttctcgatctcctcgctcttacgcttgagtccacatttttggtaggtatcaaggaggctcacagtgcttcgacgcattaggttgtgtggtccgccgaggacttgcccggtgacagaagtgctgcttgctgaggtgaccacgatgtgcccggtgcttcctgggaagacgatggtctgctcgtaaggtaggcttgggtttgggaccggcaaggaggtgctgacggttgtggtggctggctgcgacagggggatgttcttgctctggctatacactttgctgtgggagccgtacccagtcatgtcccagttggaactcggctctattttcagtttcttcacactacagaaggcacttgattgaagggtgtgaggggagaaaacttgcacatgtgaggccatacctgggagtggaactgccaggtcaggtggcgactctatgtttaaccttttgaggacctgacacttgttttccaaagtggcctcctgaagtccccaggagtcatgcaaagtcccccagaggtcccaggcaaagcgcacagaaggcccttctgcagagatgctgcccttctgtccttcggtaaaataccagcctaaattcaaagcaggagtcagggtttgtttgatttgaggtaaataaattagagaagctgtgactcgctcagtgccagcagcatgcttagcctggtatcgccccggagaaagagccagcacctggcatggcagacgagggttggcacaatgcatgcttgcttgccagatgaagaggcgctctgtgcaaagtgcagctgcagcaggacgcaaactggtgctctctctaccgtccctcaccagggcaaagctgtctgtgctcctggtcaaagcctcggaggacttatttgctgtcatccacacactgtgctccggaaagtgcctgctcagaaactggcagggagaagacccggagggagtgaggaccatgagaaatcagagagcaactagacaaggaagatatcaaaagagacgggtccttcgaggcctgcacacctgttagtcctaatatatttcagagcaagggatcagactggtgcacacatgggctgaagcccagggaaggagccaagtccaccaccaatgcaactggtgagtcagtatcaggcatgtgtcccctccaagctggcagtaaacaaacactcacacttcatgtttgggcactggactaaattaccaggcaaaagtacaaattccggccaggcgcggtggctcatgcctataatcccagcactttgaga

SEQ ID NO: 16237 - RNA, 14174 nt, Homo sapiens
  source 1..14174: mol_type = other RNA
ggaggccggggtggggcggggcgggggtgtgctctctgttccatttgttagttacaggaagctaccaaggatgcacatggtcaagtcactttctacttcccaagttcctccttataacctgagccaaacaatttcaacaatgacaatccattgccccttcagcccagcaggcgactctgacagggaggtgtgaccaccagtctcaaggctgagtggggccttcttgctggctctcgcgctttctgggagtcctgggtgccttggcccagggcagtggtgacagcagggtggaggcagaggtggccccggggacagtgaccctatataaggaagggggcggtgccaggagagattcgtttggagattggttacaaggaagcgagggagagcagaggcagagccctttttcagatacaacatacttacttttcaaatgaacaaaaggcaatttctatgttttaaaaatataagccccaaaaacaatgacacaaaattcatttggttaattcatgtaaaggaaaaaacagcaacaccaccacacaaacaggaaagtgggagtatgattaggaggggtgagatgaaaactattttacagtaacatttccaccaaaagactgtcctaagaacacgctgtcaatacagttcacagggaaaaagcaaatgtggtatttttttgtattttttaaaagctccctggtcccaggtgttttgcagttttcaaggtcttatctgctaaaggaatgccctttaggtcacagcaggtcctctgcagtttggtggtggcacaagagaaaacataaaagaaaccaagactcagggaaactgccattcccccagtctgtttctgcatgacagtggggcccattcctgtctcgaagcatcttcttgttccaaatatgatgtctgtttagagtgggtctcaatggaccaggctgagctgcccctctgtctctgcctcctcctgctcagccctgaccatctctgagaggatgctaaggtccccctcccaccgaactagactttgagtctaagctggacaatgagtaaaacgtaaacatagccttttacattgattttgcttttaaggggaaaacgaataaatgacagcagatatatggaaaacccagccagcgaccatgggaataggggtatatggtcctcccctacaaaacgctgatcaaaatatcacccccggcccagaagtagcagctgtgccttcatggtcacctgaatcccagtctcttctactgcctggtgcctggaaatcagtggatctattaataagttaaatattcaaatcaagacaaaaatcaatgaaccaggttatctgttctcaatgactcttccaagatgtcagagagaaggccttgaagacaagtgtttagacgacacgcatgagaccttcgcatctggcccgggctgcggactcacaccttttccctccatctggattgcctttcatgttctcttgagttcacgtggaaagtaataatccagagggaagtgcgcatgctggactacagaagagtctgggacaacacacttgccttgggggagacacaacctccaactaagaggcattcactggggtttgcggatgtcagttataaacagaacttttctttaaaaagtaccagtctaaatgtaaactataaaacactttaactataaaacgtagccagaaatatgcttaagtatccacagtcaattgtttagtttactcatttaaaatgtgactgttttgatagcttagaaggctaacagcattttacagtagctaaaaacatatatacttaacatgtgcatttgaacatcgcatttgagtacaacacacaaagaataatctcttccttggtttaatttttgttgtaaagatgagctattttcagaattcacttaagcaacgatgaccgggggtatgaagtaatcattattttcagcccacagagaattcatagtctttaaattccaagatcaagctggctacatgatttcaaaaaaggctaaaaccaggatgaatgcccacatttgaggtaattattgccattaggtcacagtttgtgtaagataatgtatctaaaaccttctaaaaaaaaaaaaaatctttaggtgttctgccagaattccagaatacctattgaaaccaaccaggatctcaaactccgattagttaggtttgcttccaatggagttaaagttctaaaagattctagaacttgtgtaaactacctaagaatttaggcaaacaagcctggagccagtcaacaaagaaggttttaaatgaaaaaaggaacaagaaacccactcaaaacaactgaacaaatatttcataataaatgataatagttattttaaaaaattaaaaatctagtcctaagcatttctacattctcaccatctttcaatcaaaataaaaatgcatctgtatttctgttaatctcataccagggcaagagacacgccttccttttatcatgaaagctggctggttttcctgtttatacaattgttgctatttctttgagaagagtatctcaaaagaaaacattcttttgttcctctaagtcttgtctttcttccacctctacttctttttttttttcttttttttttcttttttttaacagaaagaaaaaagttcctggacaccagacccacatatggtatttacaaatttggtgtgaaccctgcctctggttctgcccagagctgaagagtgaatctattacagagatcagagctgtcaggataattatcaagtgcagtaaaaaatagcattttgaaaaaaatatatacctttagtattgcctttctagaattaactataagcaagaaaaacttattttttaaagaagaaaagaatactttttcactcttacttataagagctggttgtagcagcactactaaagctagttggtatgctggaaagaaatctaaaaggaattctatgaatcaaaagaaactctccagagattttctctaaaaatcaaacgaattctgccccttttgcctaaatccaactcaggagccccctctttgcacagtcctttagctgagtcccacggtgcatgggatggcacagggtgatgctgtgtaaaggcctttctttgctcagacatgcaggagacagctgtggctaatggctgcaagctcagttctggagctgggcagactcaggttcaagccctcctcgcccctcaagagttgtgtggctctgggcagtttccttggctgtagggggactaatattgccgatctcacagggctacggagaagatgaaacaggacaacccatgagcaattcccagcacagtgtgtggcatgcaggaagcgggagtatcactaaatggttcatagaaatatgaggccacgcattgctattaattaaaaaaagttaaaagattaaaaatcacatctcaggaagggcctgatgaacaaaaaagggaaccttggggattctggcccatcactgctttatccttccttcaacacctgccacttctcagagcatccggtcagctcccttatctataaatgggggctgttatccccctccctgtgggatggctgttggggccccttgagacaacgctcataaaggccttagcccgggagtcatgaaagcattcaacaaatgttggctattatttacttgagagatattgcaaattttaacaaataagggacagtcagtgtcatgttcaacacagggatctgagatgaggggctcccagaggcttgggcaagtccagcggggggcatcgggaagaccctctctggtgctggtgttctgggacgggagccctgcagggggcacttctctgcaaactctcactgggtttgagggaagaacggcctggagttcttttttgaacttttcagaagctgcaacaagagaaacctctactatgctgggtccctctagtgagccacggtgccaaaagcctccaataggttttttttgcatttaaatcctgtttcaccgccttccattctctagtggcctgagattttactgagtctggtctgtggagatgagaagtgagagttctaaggcatcaaagtggaaaagtactgctattccgagcccagcccccgcgtgctctacgcccttgatgcaactgaactcctggcagccctgctttgctctctcccatggtggcctgggattagtcaagcccacgtattggtatggcaccttgtctcccgatagcagcagcatcgaaggggtcacctccactcctcttaaaagaatagcacagttttgaaataaatgcattttttttttttaaaaaaaaggacagagaggaaagagaaagacaaatagaattgcatcactaatgatgtcattattgcctggaaaggaacgaagggaaggccattttgtccatttctggaggcgtctttgagaagggttctttggctaaagaaaggaacagtttcaccttcctttccaatttggtaaggacatctctggcctgctcaagtttgaagcttccccatcagaagtctgtaaaacacaccagaaggaaaagacacagacagggaatgaagcctgcaaagtccctggggctggaatgtcttgtggccaagtcactcctgctggcgctgtggagtcccaggctggcctgcagaaggaacccttacctctcctcaattctctctgctagttgagagcaccgagccatttccttctttccattttctgtcctagggtctacttgacaggccaacaagagtggtggtcccacaccccaccctgccctcagcatcagacaaagagaacctgggacaaaagctggggcgagctgggtccccacgtcgctctctcaaccatgagccatcagtaatacttcccgaagcctcctcatctcctccctccagtttccaagaaagtttgttccactcactcacacatgctcacacggcctaaatcttccaccccaagcttgttccaatatgagtgtttgccattcccaaggtccaaccaagggaaatcgttctgtcagcagttgggctaatctccccttcccttcctgatgtccatccgtctcacacgttggtgtctgggcgggctgagtcttctaggttgaagaggacaaaggtcagctggctcccccagcccgtgaacacctcagccaccaggaagactagaaaggctaacagtccaggagatgaatgccgctttgctccaacccttctttttcctctgaattccactgaccgcacgctccacttcacagtattaactggcatcaagcctcgactctcccaccccttgatctgctcacccacttcccttggaaacatccaaaacatcatgaagaggccctaagcacagagacatgggggcccacgtccagacgggccagtcagaacccagtgagcagaagcaaattgccctgcggttcaccaggctccagttaaacactcctccgtgacctgacatttcaaatcttcccctcttcctctgaacaatgtctcttcaaatgggaaggagggagcccacaaaagactagaggatgctctagatgattcgtgggctaagtaaggactaggttggcatccctctgcttgagagcttggtcctagtgacagcagcctatttgctaaggtgactcaatggcagattcggccaggtatgcaattgggcatccagggagctggcctctcctgcagggagcttctcttggggcttctgatgtggcagctccatgcatgggggtagaggaggccattgggtgaggactaggagaatgtgcactaatgtttgctgagcgtctgtggggctggcatcgcccaatacttcccttcccttcccttcggtgaagctggctatttcacccctttcttcaactggggcctagcactttgtgggtctggggacagcgtgtgagcacccagcgcacacagcacagtgcactgaagatgtggccggagcccagtggggatgctttcagagggggtgcagcctgtgatgcctgagcagccgcccagctttgttcagggtttctctggcctcctgctgtccctccacccacttccagctggctagaattgggtgctgggggcatgcatcacagggggagggggcaggctgaggaactgggtggtgtggtgaaatttcctggggaaggtaccacctgccagtcactcttacgccacctcactgtgcccagcagcttctgggagggggcaaatgtccctgcattgaagaacctaagccacgccccaggtgcgccgatggcaaaaggatggattgtggggaagcggatggggtcacctctgggagggaattttcttgcttaaataccagaggcaagccaaagatttagttaacagatttcagaagcacaggagagctctgaggatgtgggagagaagctggctaagggctggacagtcagtgactcgacattccccgagcccatgagatgccacctgacgtcgcatcccaggcctctgggatctagaaaatgacaaccttgatggtgaccatgttgtcagaagcccaatcaaggctttgattcttctttaaacttttgttctgtggtggatctttcttgacgtctcttgttgggatagagatgacagaaacaattttcctacttcctaagtctttcctttttttttttgcctgacaaaactggacatctggatgtccctccagtctacttatatactcacagagagaataagtttaaatattaaagagaaaacacaaagatacttggaataaatgtgcatttaaaaccctgactaaaatatcaacataatgatcataattacaatggtaataaaaataattagtacaataatattatctttatgagcagcatggaaatttcattcctgatctggaagaataaaaggaaagaaaatgtcaggtgaaagagtaagtagcctccaacttaagcagacagaataattttctttaaaatgaaaagaacattttaagctgtctttccccctaaaagatcagatctagaaagggctggaaatgaactgtgcccaggaatctgggggtgctctccagtaaggcgaactgaggctcatttgcagccaagacttggaactcgggatgagacctaatgggctattgctgccatctggctgccaaaaagtccctaatagatggattttccaggctgacccagctgtggggcgggggggggtcctctggcttctgtgtcctctgaagcgtttgctgccctcaccctctctgaactgaccattgtcctgctgtctcagagggctgcgcttccccacctccagataaagacagtattgataatggcccgagggaagggaatctccttgctgcaggcctcttgccggcacagcctccagcaggcacttggcaagactgcccggctgtgcccagcatggagcagtcatggtgtccttccttctcgctgaggcctggactaagctgtttccagtttggggacctgtttctttataagtaagaatttatggttggggtggggaagtttccagagttatttcacagctaagagctaagtaacgacttcgttactgagttaggttggatatcactacaaacacacctttcacagtagatccttgagggagactgcacagtgaggaagtaaagggagggaggatgaggatggggccgctgactcgggaaagatctctttgcaccttggaaacctgcctgtggggtcagctaaagactcaacatcagaagcaaacaattagaaccacccttttcggccccatccttggccagattctcctgccattcacattcacatatttcagagttatttactatgaagagagggaactccccacttctccacacctccatccccagaagtgtccaaagcctgagaaaacttccagaatgtatcaaaggtgcaaagagggcaaagggcagatttctttggaaattcaactgtgtgagtttttccaaagtgcagcgtcagacccccggccaccctcataagtgtccctccaaccttctgcccactagaaccctcagaaaccaaaaccaaaatcatgtcttgagcagacctgggtaatgtgaggagagaattcaacagcaaacagaggttggtggttgtctacagagggagggatctggcaagatcgttagagcaaaacagcccagggagccggaggagagagtggagccccgggcgaggctgagagctccaggctctcgtggaggcgggagggactgggggatgccgcctggggcgggagacggctgcctggcgaggccaacagtccggaaacctctggcctcacaaatggcggaactggggacagagtggggcaggggtgaagggtggggagtctctctgggcctccgcccacaaattacaactcaactactgccacaactcaactcccgccgtccccatctccagacgcacccgccgggcatctgtctcccatatttctttcgagatccacggactctctcctagctcctgctggcttccctggcatccttccgctagcaaacagcccaggaaagacaacgggcattaacattttaaaaagaaaaagaaaaagaaaaaaaaaaggccagcgtaaactgttacaacagcacaacagaagagctgagattgtgtctgactagcctcagtttcttggagtaccagtggaagtaaaccctcacgccgcgtctgtcgctcggtaaggcactaggagggaaggatgcagtgtcaagactgcgccagctagggtggcggcgccgagggccacgcggggagggcggcgcgtgcacacccacacgtgctcgctcacccgcacacctgcaccgccacattggttacatgcctatgttatatcgcttttttttgtgcaattacattgaggaatattctattggtatcattggagttgaacacaaggtaggagacaagggtgctgagtgctacattctactagggtgtctgtgacgaccgctagccctacgctacgcgactaggggtggattcaaagagaaaatacattttcagaaaagaaaaaaacctaaagtttgcaacacacattattaatgacatttgagaaacaacgttgcttagggatttatccagagtgctcagaaaaagaaaactcgccccgcgcccccgggggccttccagcagcctggccgtcccccgtctttcctgactagggagcccggactgggcttcgccaatcccacaccagctccaaacatcagcctcctcaggctgcagcccgacattctggagggctgttgaccctttcgagttctggaaaaatccctaaatcttatgttcaattaattaaaaatctatttgatttccatatcaggtgtccctgacagcagtcttccgtatcacttgctgccatatgaaaataatctttgaaaagttcataaagttcttcaaaaactggggccccccgtttctggaatcttcctgttgctctcttctcctttccagtttggcgtagaatgggttcttgagctgggttttttgttattgactttttttttttcctttttcttttttaaaataaaaaccatagatttcccaccctctttaatcccttccttttaaaaatgttctcttctctgctctacgtcctcccacttcccggttcaagtttcactggtgtcccgacccgtccccctgccctctgcccccccccccccccccgcccctgccccgtttgcattgtttgtgtgcggcatcttcagtataaaaggccagcgcccacggtcccaggagcgcctccctccttctctccctcctccctcgggccattctctccctccctccctccctccctcccctccagtgtttatatgtaagggtactggttgaccttggcggggctcagtgggtatccagtgtagacggtggaggctggcgaggcgctgatgtaggtctggtgggcaaattgggctggatactgactcgggtggatggtgggcgagggcaggacccgggggcccatgctcacggggacctggtggacgatgctggctgggtaggcagtgtgctgcacggtgtggcgcgcagagccttgcgaggccaccaggtgggccacggtgccggtggagcccagggccgccggcgcagtgtaggtgtagaggtggggctgggtggggaggtgggcagcggcagcggctgcagccagatgcgggtgcacagtgccgtggctggggctgttgtgcgggaaggagtacggagcctgggccatggtgggagtgatgtaggcctgctgccttcggtggctcccagtgcggtccgtggtgatgtgctgctgagcctggctgagattgagtggctgctgctgctggaagtgggggcccggccgctgctgccggtaggtgatggctccagatgagctccctgaagagtgaccgctggtggaggtcacgttgctggaggacttggacttgtaggaggacgagtggtgactggtgttgactggcaccaggctatcacactccaccaatacttcgctggcctgggttttcaggggtggcacgatgatggttcgggggttccccgtgcagtgattctccaggctccccttggtgtcaaaggcattggcattgttgtgcccagcacgctgctgcacggagtaggggctggtgttgctggaggagtcggagtagggggagtcgtggactgtgacacagctgatgacgttttttctttgcttggagacagtgctggtgggggcgtgtttctgttcctcctcctcgtccgtgtcactgctgatggtgatgacgctgaccgtggggctgggagtgtcgggaatgacaattgtctgccgctgccgttcccgggtggtgctggaggccacgtcgccccacccacaggtgaccgaggtgctgcaggccgggctactgtgcaccatggcacagcggggaggtgtgttctccttgacacgcttggatcgctgtggggagctgatggcctgagaggaggacacctcacaggtggagacatttctcacagatgactggtgctgcttactcttccgggaggaggtggtgctggttggctgctgccgcatcacgtgggccacacccacatttaagggctgtgctgctggaagggtcacatgaccggtcaatagtgcaggctgctgcatgatgggattataatggcttccgtgagcatgcgtatttctccagtccgccagctgctgggtgcctgccatggtctcgggaatcacggtggcatgctgcactgatgtgtgggtggccactccagtcagttgctgccatgctgggggaagcaggatctgctgggtcccacttggccaagcctgggcaagcagacctggttggatctgaagaggctgagctcctggggcttgagtgacgatgggaactgcattttccattcgcaccgagtagccagcgtgcttagagggagaggcctgcaagccttggaagccggggggacacacgatgagagcttgctggaacgggtcaggccgggcacaaatctgggctgttcctgtctgcaggggcatgctccgctgggccactgcagccatggatgccgctgagggctggttgtggacagtggtcagctggttgttaaaggtcatggtcaggttggtggacgtgctgggggccacgtgcgtgatgaaaggggttttgctctggttcaccgtgtcatacatattcacccgacgcttgcagatctccatgttctggaaacatgatttgacgtgtgtgctgtggggaaaatcgagtaagtgtgtcatggtgacaaagggatggttcagggtttcgattggagtgattctcttgtcagcatcaatggtcagcatcttcttcaacaggtcaatgaactcccgccggtcagccttttctaccaacatgtcgctcccttccaaatctgtcgtcatgttcacctgggccatatcatctaaacagttgaaaatgtactttcttgcttcttttgacttaatccctgtctctgcttcatggtcatctggtgtcttcagtctccacaaaggatatggtgagtccgtgtcacggttgaaaaacctagttgtctttgtcccggcgcttaataaatattcagcaggcaaaccctgtgtttgtgaaatataccgaatctgatcatactccgaagctcctggatataacggccaacccaggaacaattctgcaataacacagcccagggaccacatgtcaattgcctcacaaaatggtaaaccaaggatgatctcaggggccctgtaatatctggactgcaagtaggtggagcacacagccttggagacgtggctggctgaaccaaagtcgatgaccttgactctgtatggttgtctagatggatccaccagcatgatgttttctggtttgaggtcagcgtggataagacctaggcttttgagtttcatcagggctgtggctacctgctggagaactgggcgaatgtatttgaggggcaaggggctaaacttgttttgcttcagaaagtcatagaggttctgctccaacatctcgaagaccaagcacgtgtggttcttgtgctggaagcattcgtaggcccggacgaagttatagtcatcggcactctccgtgctcaaccgggccaggatgctcacttcaatctgaccttgtcgggcataggatgggtggttcttcaggatcttgatggctacgatctcattggtgccccgtttccagcacttgaccacttgcccaaacgtccctcggcccaagaactctaagacctcgtaggtgttggtcatggagcacagcacctcatgctgcaccagctgatagtcgccctcgctgttggagccgctgtttttggaggtggcagtagacgtggtggcagtggcgacagtggccccgcttgcattattctgaatcatgggtggatgctcctcgatgatctgcacgctgcttgtgttctcgatctcctcgctcttacgcttgagtccacatttttggtaggtatcaaggaggctcacagtgcttcgacgcattaggttgtgtggtccgccgaggacttgcccggtgacagaagtgctgcttgctgaggtgaccacgatgtgcccggtgcttcctgggaagacgatggtctgctcgtaaggtaggcttgggtttgggaccggcaaggaggtgctgacggttgtggtggctggctgcgacagggggatgttcttgctctggctatacactttgctgtgggagccgtacccagtcatgtcccagttggaactcggctctattttcagtttcttcacactacagaaggcacttgattgaagggtgtgaggggagaaaacttgcacatgtgaggccatacctgggagtggaactgccaggtcaggtggcgactctatgtttaaccttttgaggacctgacacttgttttccaaagtggcctcctgaagtccccaggagtcatgcaaagtcccccagaggtcccaggcaaagcgcacagaaggcccttctgcagagatgctgcccttctgtccttcggtaaaataccagcctaaattcaaagcaggagtcagggtttgtttgatttgaggtaaataaattagagaagctgtgactcgctcagtgccagcagcatgcttagcctggtatcgccccggagaaagagccagcacctggcatggcagacgagggttggcacaatgcatgcttgcttgccagatgaagaggcgctctgtgcaaagtgcagctgcagcaggacgcaaactggtgctctctctaccgtccctcaccagggcaaagctgtctgtgctcctggtcaaagcctcggaggacttatttgctgtcatccacacactgtgctccggaaagtgcctgctcagaaactggcagggagaagacccggagggagtgaggaccatgagaaatcagagagcaactagacaaggaagatatcaaaagagacgggtccttcgaggcctgcacacctgttagtcctaatatatttcagagcaagggatcagactggtgcacacatgggctgaagcccagggaaggagccaagtccaccaccaatgcaactggtgagtcagtatcaggcatgtgtcccctccaagctggcagtaaacaaacactcacacttcatgtttgggcactggactaaattaccaggcaaaagtacaaattccggccaggcgcggtggctcatgcctataatcccagcactttgaga

SEQ ID NO: 16238 - RNA, 3538 nt, Homo sapiens
  source 1..3538: mol_type = other RNA
ggatccgagtcacggcaccaaatttcacatttcactcatgtactgtgcttgagtgaacaccagtaagtgtcgtctggtgcaggcagagtcatgggcagaagggcagaagattcctgggacccctgttttcttgccttcctgtggagtggatcagacagatgcagatgggcaaatctagagactccacctcttagttgttctttccttagcaactcagtagaagagcctgttctcttcctcaatgcctctgcgaaagcatctggttcactcccattaatctggatttagtagcatatccctgttggagccaatcagttggacagagagaagaaatatgcactttatcaaggcctatgaaatgggcccccgcccttggaaatgaagggtgggttagcatggggaaaaaagtggttcccaaaattaagaggaatattatcaggaatactggattctagcaggaatgccacaaatgtctacatcatctaatttttgtttctaattcagaattctagattacctcccatctccgatttgctaaataacaatctgtaggggtcaagccttaaatagttgaatttgtaacatctccacaatggtattctaactcacaatcagagtgagagccattgcaacccaaaagagtaatgctataaatagggaattttatgcatcctgaggccagtgagttagacagtcaaagataaatgaataactgcataatttgtttacacacaatggctaatgtatataaatctactgttaacaaaatcccaaaacatgaatgataggatgcaaactaagttaatatatatatcactgtcgcattgacctaagccattggaataactattgatagttgatgctcatcatctgaacatatcaaaattttaaacatgacagataagcttgaatgaatgcaacaaggaggtattggtattgtttccctttctgctgttaaccagctatggtcaagtcacttcagtggctctcagttctcacacctgtaaaacaaaactgccagatttactgatgtccaggtcttttctagctatgatattttacgattctatgattaaactgtgatgccatacattgataattttatcaagagtttcatctggactagagctttgaaattcaaagcatggcccatggaccagcaatgttagcatcatatgggacctatttagaaatgcagaatctaggctccatctagacataatgaattaaaatctgccttttaagatccctaatgactcttatgcacattaaaatttgagaaacattgatcaagacagtagtttcactttggactgtggttctgaaattacctgagagtttatttaaattgtagatctctaaaaatttccttgtcatgagagacaaattaataacatttgagtagtagctcaggaatatgttttaaaatctccccagataattctcatgtacagacacatcagtcttatctagcacatcatcaaatatgaaacacgctaacacagccaaaatcttactcaaatctccaaatctgcaaacttcaccattgataatctataaaaggtattatttgcaatcatttgtacttctgtctggtttatgtacacatgggaaatgatatctcatttatagatggagaaaataaaattcgaagagaaaaaatgaattaacctgagataacaaatttaatggcaaaaatgagattaggtagatatcatcttagtatatttattttgaaaatttttaaggatcattagtatacagtgttgaatctattattttttctggaaaaagttcagcttatcttaccaagtaatcaaacacgataaaataaagatccaaaataatttacatttatgggcttcaacatctctgaaagaaactgttcttaatatcttcttatcactgtatctggagtggttgcccattaagtcatacacatactaggtgcttcaagggggagagagtattcctttttatagtcttcattaatggtgagtagtacgctttccccagaaatatttgtttaccaatcaaacataaaaagttttagaaaatcaaagaatatacagatatttacggataatctggaatatttatctaaaatattaataattcagcaaacagctgtgtttggcattatttaattagccactaaatagataacaagatttgcttgttcatctgttacaattaatctgttgtgctctaataacaattggcagattcttataaagattctatgtttaagtgaataaataatttgtttttttaatattaaaatgggaaataatgtaagaaggcattttattttatctggtgcttgtgaggtatctagagaaaacataatgagaggcattctttgaaatacacaacccttataataatttaataaagagaattgtcatcttaaaagaatcaggatgattgccttgatgacagagattattcttttaacttcctgaatctgccatttgaaaatcttcaattgataacattttgaatttattaacagtttgccatattaatagagaaaaattgcatgctttaaactggccatgtaagtcttagacaaaattacaaactatctgtctactcaacagcaagctttggtatgatcataagtagataaaaacgatcataagcaaaacacatgtaatataacaaaacaatttagaaatacgtcactacaaaatcagctcattcacaggaatcactgatacaatctattttcactgatttttgttccattggttgctgctactaccagccttctcattttgaatgcctgtggcctttcttcccagttacatatggaagttgagctcagagagtctggggaaaatgtattggcctgatgattaccattggcactgtggtagacatagaccttatgtaaacattttgacagaattaaacggcctcatgaggaggaagaaaaactaatgaagtgaatcttcacttggagtttggtgaagttttagagattacaccctttgagtaattgtatgttcctatgggacattcagcacacgtcatgagaacaagaaaattctccattatacttgaaaactctaacttggactaccaagaggatcattaaaatctatccttgtcctctcaaatgtccagcataaatatatttagtaaatggctaaattttgtaatttctgcatgtagaataccataaatatagagacaagtgttataagacaaaatagaatgtagattatcctaccctaatcattaataaggaatgctagagaaatgtaataatattaaatctgcagaacaaagggaatagaaatttaaagttccttcctttaagctcggttttaaatcttgctctcaatttttttctgttgaaatagttatattttattaacattttattataggcataatatacttacttatagtttatctagtttttgtatgagcatctataaattttgaaataaagcaatgttaaaaacatgcttaatgtccttaatataattacaatttagcttttcagtgctctagaaaaaacagtaca

SEQ ID NO: 16239 - RNA, 848 nt, Homo sapiens
  source 1..848: mol_type = other RNA
ggatccgagtcacggcaccaaatttcactgtgctccagcaggtcctggttatccttgggacaattttctaacatggatccatgcctgatgcactgtaggcccctaatagcccagcttctgtccatctgtaacacatttgctgctacagattgtgtctgtatagagaagagagaagacgcaaagctcttcttccagtccttgaagtctgcagcctgggtgtctgcagaggacaatgccttgttctttaagatacccagcatggcactgcagtacatcttgcaatgggatggcctcctgtcccaggctggttcatgcctttcatcctgagttgctgggacaggctccagccgcctgtgacccttgtcttcatgcaagttgccgacttgttggaattcagtccaattttcaggagagggactgttgctcttataaacagaggtagtaaagtgcagcagggagcagttccaggcgcagctgcagagaaaaaagttcaaagagaactcggtagcctcttggaggtttctatgctgtttatcttttttcaagcaaagggaagtaaaaagcaataggagaactttctttaggccactgtttccatgagatcgcattcctccacacgagggctcttcaaaaaattgaagatggtctattttacaattaaaaattaacttattaggttaagtgtttataattcctttaagaatttccttggagtaagcagattgagaaacttccccacttttcaactcaggtgttttccactcataattttctttcaaaatggattccgtgaattttcttaggccaaattgtcacctcctttttaatgataccaggcagaaagaatt

SEQ ID NO: 16240 - RNA, 129 nt, Homo sapiens
  source 1..129: mol_type = other RNA
ggatccgagtcacggcaccaaatttcatccgtgtccctgtgaagagaccaccaaacaggctttgtgtgagcaacatggctgtttatttcacctgggtgcaggcgggctgagtccgaaaagagagtcagc

SEQ ID NO: 16241 - RNA, 179 nt, Homo sapiens
  source 1..179: mol_type = other RNA
ggatccgagtcacggcaccaaatttcatgcgcgtccatgtgaagagaccaccaaacaggctttgtgtgagcaataaagctgtttatttcacctgggtgcaggtgggctggtttatttccatattaatgcttgatatctaatatggcttgttaacatagcttaccatattttctgggcat

SEQ ID NO: 16242 - RNA, 129 nt, Homo sapiens
  source 1..129: mol_type = other RNA
ggatccgagtcacggcaccaaatttcatgcgcgtccgtgtgaagagaccaccaaacaggctttgtgtgagcaacgaggctgtttatttcacctgggtgcaggcgggctgagtccgaaaagagagtcagc

SEQ ID NO: 16243 - RNA, 111 nt, Homo sapiens
  source 1..111: mol_type = other RNA
ggatccgagtcacggcaccaaatttcatgcgcgtccgtgtgaagagaccaccaaacaggctttgtgtgagcaataaagcctttaatcacctgggtgcaggcgggctgagtc

SEQ ID NO: 16244 - RNA, 124 nt, Homo sapiens
  source 1..124: mol_type = other RNA
ggatccgagtcacggcaccaaatttcatgcgcgtctgtatgaagagaccaccaaacaggctttgtgtgagcaacatggctgtttatttcacctgggtgcaggcgggctgagtccgaaaagagtc

SEQ ID NO: 16245 - RNA, 36 nt, Homo sapiens
  source 1..36: mol_type = other RNA
ggatccgagtcacggcaccaaatttcatgtgcatct

SEQ ID NO: 16246 - RNA, 173 nt, Homo sapiens
  source 1..173: mol_type = other RNA
ggatccgagtcacggcaccaaatttcatgtgtgtccgtgtgaagagaccaccaaacaggctttgtgtgagcaataaagcttttaatcacctgggtgcaggtgggctgagtctgaaaagagagtcagcaaagggagataggggtggggcaatttataggatttgggtaggtaag

SEQ ID NO: 16247 - RNA, 1918 nt, Homo sapiens
  source 1..1918: mol_type = other RNA
ggatggaggaggggtctgcttggaggagaaaggagctatcatgggcgtagttttaagtggatctatgctgccaaagataggcttgaaggtaggagttaaggtaccctgaattgtggaaagggaagagattgaagatgctgcagctgtgactgaaattctggaatatgaggagcttccaatctcgctgttgtgcaggggccccaaaatcggttttaacatgaggtgagcagaagttgcatcaggaggtgcagatgcagaaagatgggatgttgggctactcaccattccaagcaaagtactttggatggtgggtggtgcaggtgggtctgggggcatgggagacctgtcagcctgagaggttgaaggcggccaggtggtgtcagtaactggtaatgtgggagaggtgggggtcagcaggatgaaagtagctgtgggctttgagtctggagaggtgcctggaaggagctctgactgtgagcacccaggtggggtcggtaggctgggtgtcttcaaaggagaatgggccacactggttgcctctcccgtggactgtggagaggccagtggacctagagacttctgcatttttcttaagttttccaactgaggatttgctccctgggttagatctgtttctgaagaaggcagagcaagagacaaggaaggctgaatagcaagccaagtctcagggaaagggtctgtgttgacctcagttgtatcttctcctgcgttgttgcttacctgtagctcagctttcttccccaaagtcaagttctcatcagagactgcataaccaagctggggaggtgggatctctgacaccaggttctcagggctagacggcagctgtggaatcttctggttttgctgcccagaactttcagatcctcctagggactcaaaatctgataccagtgggactggagaggaaggccgatgacaacttttttccttttttattggccactctggtgtctcgaatgatacactgggaacacttctcttccaagggtctgagaaatttctgcaagagctgtaagagctgccaatagcattccttttggagctgagggtgccacctctgtatatgctggccaaggagctcatggaggagcaattgggcctcttagtcaagctgtgatctgagccccaggagtggagacttctcttcagcggcccaggcctgggcacaaaagaagtgagggttccatttttcatcaggggcttaaatgccgatggtctggtctctggactccttctcttactgtccagactctcagggaatagtggttcttccaacctccctttcccttttctgcactctctgagggccctcaacactgtctcctttgaacatggatctgcgagctcctcagagggcgggagtcctgcaagggcaattacatcttcaggagaagtggaagggggcactctctggtcaggaggagtgatcctgatggtcactgggctccaaattggcctgggatgtcgaagagaccaaatagtccgctttaagtaactttcccaccagtctgaagggagaggccccaggggggaattctgggacttcttcatgggaaagcgcctccaggcctcgttggccagccacgtggttggattggcaggatccaggtttggccgcctcctcacaggtctataccgtggggcagggtgggcgcggtggacgaactgaacccgatgaacttggtgaaggggctgaggtggccggcgtttcgtgggcctctcgggcaagtcggtgcgcacctgggctggggacgagggcgaaagttccagtttgctcaggaaactgcccatgaggagagatgaggcgcgggcagtgagttcaagcacggttttggcttccgaggtttcggacgtctgcagaatcggacagagtcgaagagcgcagtgttcggtt

SEQ ID NO: 16248 - RNA, 45 nt, Homo sapiens
  source 1..45: mol_type = other RNA
ggcaggttctcaccctctctaggccttggtttctccatctgtgaa

SEQ ID NO: 16249 - RNA, 2612 nt, Homo sapiens
  source 1..2612: mol_type = other RNA
ggcaggttctcaccctctctaggctagggaagcaccctattctatagcacaaggcagccatacagagttttaggccaaaaaaaaagaaaaaaaaaatggggctttgtcagcaaggaagggagaacgaaatggctgatgggtaggcatatgaatgtctaacaaaccaacttatttgaacccagctttttcacacacacaattctcacacctgttttattttgaagttctctattgtgttctattttgatctacttctgtgtcattagctattcctgggtcattatgacttttaataaactttatacatgtatatttggtaggaactttcctaaattttttcaaaattaaaattttttccccaaaacatgtgagaattaggattgcagtcatgcattgcttagcaaaggggatacattctgagaaatgcatcatcattaggagattttaaaattgtacaatcacagagtgtacttacacaaacctagatggtatgatctactatacacctaagctatggcctattgctcctaggctacaaacctgtacagcatattattgtagtgaatactgtaggacactgtaacacaatggtaagtacttgcatatctaaacataaagaaggtacagtaaaaatacagtattgtaatcttatggaaccactgccatatatgaggtctgtcactgactgaaacatcattatagggcacataactagaatttaataaatcaagttaaacaaattatctttgtaatactgtacccttccatgaaaggaaaatggtatgcttctaacttgagttttctttaatgtcctaaagtacatttttatagtttttattttgtgtttttaatataatgtttggtatagtcaatcttcttaatctgccatttctatggcagagtacccagtgaaacatcttgtttggtgtgtcagtcaccccctgctgcagagttccctgtcacacaaatacatgcaaaagggtaataaataaatgggaaacaaagtatagttttagtaatcaacatgcaagattctaacaaaagctggagataactgcttatgccagataatttaagtaagagaaagtaagtagaagaggtggtaagaaagatatatcagatgagcactgaccccaaaccactaagatgatatggtccaaagaatgtcagaatgactaattcaattatccaactctgctcagctggaagaggaaagaagggaataaagatgttagatcctttaccaggacttccatgcacggggagagaagttgaaagtcaaaactgtaacaggaataaatacaaaaattctttccaaacatacctaatattctttggccctagagtcactgaattcacatttaaactaatctatatttcattttgattacattaatggagctctgaaggaatgaaacctattaaagaaaaattaaatttataaacaatttaggcagtcatatatgtatttatatatacacacatacaatgtatatatgaaatccttatacaggtgtaaacattcttaataaattataagcaataaaataaaaaaaatttagtatgtttgctttttaaaataaaacaaattcatactttatcaaaatttgttcattcttctcacaaataattctgttggtacataattttctctcatgctaattcaacaaaccctgagctttgtttctccatctatggctaaatacatatcactctaaccaaataaaaaggtttaaaataagggccctgcatcttggtgtctggttatttgaaatccggttttcattttgaatagttttggttaagtgtatgtcatggcagaatgtcccttcatctcctttgatctgtgttaaattgataaaaatacatgcttactcctgtacaaacatcgaacaatgtaattaaatcatcactacttgaaatacttttacatgaataatttatctctttacactgttgaagccttgcatttcagtatgttctacagcttctgtatcatcacctgaaatttgcaagcaggcattgaagacacttcagctgttacaatactttttattcccaagtttgataagccacctctgattaagccacacgtaaatgctaaatactgatgatttgtccttagattgtcgatttgtttcttgaataccgtagtccaaaaatctttacaaatgaacttcatgatatctaactcatccttgaaccttgcagtatcttttgtaaacctttctatcaatccttgtcccactcgaaaccccatgttttccagcttagtaatacatcgtccgttttccacctccccctgctccgcggacttgtacactccagacaccatctcgttatggagaagcaaaaacaacgcctcatccgccatttcctgctaattcttccaagcttcgagttttggctcccgtttgagctggtctgggggttccagctcgcgcctcagcgacttcgccggcgccgcggctccgtcaggccgccattctatccctgtggctaagagaccgaggtattcacacgacttcccaaaggctggtactgaaatgagtctggtactggagagagcccacacttcggggctaccaaatcctagggccgaactaaagtct

SEQ ID NO: 16250 - RNA, 2696 nt, Homo sapiens
  source 1..2696: mol_type = other RNA
ggcaggttctcaccctctctaggctagggaagcaccctattctatagcacaaggcagccatacagagttttaggccaaaaaaaaagaaaaaaaaaatggggctttgtcagcaaggaagggagaacgaaatggctgatgggtaggcatatgaatgtctaacaaaccaacttatttgaacccagctttttcacacacacaattctcacacctgttttattttgaagttctctattgtgttctattttgatctacttctgtgtcattagctattcctgggtcattatgacttttaataaactttatacatgtatatttggtaggaactttcctaaattttttcaaaattaaaattttttccccaaaacatgtgagaattaggattgcagtcatgcattgcttagcaaaggggatacattctgagaaatgcatcatcattaggagattttaaaattgtacaatcacagagtgtacttacacaaacctagatggtatgatctactatacacctaagctatggcctattgctcctaggctacaaacctgtacagcatattattgtagtgaatactgtaggacactgtaacacaatggtaagtacttgcatatctaaacataaagaaggtacagtaaaaatacagtattgtaatcttatggaaccactgccatatatgaggtctgtcactgactgaaacatcattatagggcacataactagaatttaataaatcaagttaaacaaattatctttgtaatactgtacccttccatgaaaggaaaatggtatgcttctaacttgagttttctttaatgtcctaaagtacatttttatagtttttattttgtgtttttaatataatgtttggtatagtcaatcttcttaatctgccatttctatggcagagtacccagtgaaacatcttgtttggtgtgtcagtcaccccctgctgcagagttccctgtcacacaaatacatgcaaaagggtaataaataaatgggaaacaaagtatagttttagtaatcaacatgcaagattctaacaaaagctggagataactgcttatgccagataatttaagtaagagaaagtaagtagaagaggtggtaagaaagatatatcagatgagcactgaccccaaaccactaagatgatatggtccaaagaatgtcagaatgactaattcaattatccaactctgctcagctggaagaggaaagaagggaataaagatgttagatcctttaccaggacttccatgcacggggagagaagttgaaagtcaaaactgtaacaggaataaatacaaaaattctttccaaacatacctaatattctttggccctagagtcactgaattcacatttaaactaatctatatttcattttgattacattaatggagctctgaaggaatgaaacctattaaagaaaaattaaatttataaacaatttaggcagtcatatatgtatttatatatacacacatacaatgtatatatgaaatccttatacaggtgtaaacattcttaataaattataagcaataaaataaaaaaaatttagtatgtttgctttttaaaataaaacaaattcatactttatcaaaatttgttcattcttctcacaaataattctgttggtacataattttctctcatgctaattcaacaaaccctgagctttgtttctccatctatggctaaatacatatcactctaaccaaataaaaaggtttaaaataagggccctgcatcttggtgtctggttatttgaaatccggttttcattttgaatagttttggttaagtgtatgtcatggcagaatgtcccttcatctcctttgatctgtgttaaattgataaaaatacatgcttactcctgtacaaacatcgaacaatgtaattaaatcatcactacttgaaatacttttacatgaataatttatctctttacactgttgaagccttgcatttcagtatgttctacagcttctgtatcatcacctgaaatttgcaagcaggcattgaagacacttcagctgttacaatactttttattcccaagtttgataagccacctctgattaagccacacgtaaatgctaaatacttagatgcatgttctaaatactgttttcctgcagacatctgagtaagcaggcgaaatttgttgtcctgaagtacatagatgccctgatgatttgtccttagattgtcgatttgtttcttgaataccgtagtccaaaaatctttacaaatgaacttcatgatatctaactcatccttgaaccttgcagtatcttttgtaaacctttctatcaatccttgtcccactcgaaaccccatgttttccagcttagtaatacatcgtccgttttccacctccccctgctccgcggacttgtacactccagacaccatctcgttatggagaagcaaaaacaacgcctcatccgccatttcctgctaattcttccaagcttcgagttttggctcccgtttgagctggtctgggggttccagctcgcgcctcagcgacttcgccggcgccgcggctccgtcaggccgccattctatccctgtggctaagagaccgaggtattcacacgacttcccaaaggctggtactgaaatgagtctggtactggagagagcccacacttcggggctaccaaatcctagggccgaactaaagtct

SEQ ID NO: 16251 - RNA, 2813 nt, Homo sapiens
  source 1..2813: mol_type = other RNA
ggcaggttctcaccctctctaggctagggaagcaccctattctatagcacaaggcagccatacagagttttaggccaaaaaaaaagaaaaaaaaaatggggctttgtcagcaaggaagggagaacgaaatggctgatgggtaggcatatgaatgtctaacaaaccaacttatttgaacccagctttttcacacacacaattctcacacctgttttattttgaagttctctattgtgttctattttgatctacttctgtgtcattagctattcctgggtcattatgacttttaataaactttatacatgtatatttggtaggaactttcctaaattttttcaaaattaaaattttttccccaaaacatgtgagaattaggattgcagtcatgcattgcttagcaaaggggatacattctgagaaatgcatcatcattaggagattttaaaattgtacaatcacagagtgtacttacacaaacctagatggtatgatctactatacacctaagctatggcctattgctcctaggctacaaacctgtacagcatattattgtagtgaatactgtaggacactgtaacacaatggtaagtacttgcatatctaaacataaagaaggtacagtaaaaatacagtattgtaatcttatggaaccactgccatatatgaggtctgtcactgactgaaacatcattatagggcacataactagaatttaataaatcaagttaaacaaattatctttgtaatactgtacccttccatgaaaggaaaatggtatgcttctaacttgagttttctttaatgtcctaaagtacatttttatagtttttattttgtgtttttaatataatgtttggtatagtcaatcttcttaatctgccatttctatggcagagtacccagtgaaacatcttgtttggtgtgtcagtcaccccctgctgcagagttccctgtcacacaaatacatgcaaaagggtaataaataaatgggaaacaaagtatagttttagtaatcaacatgcaagattctaacaaaagctggagataactgcttatgccagataatttaagtaagagaaagtaagtagaagaggtggtaagaaagatatatcagatgagcactgaccccaaaccactaagatgatatggtccaaagaatgtcagaatgactaattcaattatccaactctgctcagctggaagaggaaagaagggaataaagatgttagatcctttaccaggacttccatgcacggggagagaagttgaaagtcaaaactgtaacaggaataaatacaaaaattctttccaaacatacctaatattctttggccctagagtcactgaattcacatttaaactaatctatatttcattttgattacattaatggagctctgaaggaatgaaacctattaaagaaaaattaaatttataaacaatttaggcagtcatatatgtatttatatatacacacatacaatgtatatatgaaatccttatacaggtgtaaacattcttaataaattataagcaataaaataaaaaaaatttagtatgtttgctttttaaaataaaacaaattcatactttatcaaaatttgttcattcttctcacaaataattctgttggtacataattttctctcatgctaattcaacaaaccctgagctttgtttctccatctatggctaaatacatatcactctaaccaaataaaaaggtttaaaataagggccctgcatcttggtgtctggttatttgaaatccggttttcattttgaatagttttggttaagtgtatgtcatggcagaatgtcccttcatctcctttgatctgtgttaaattgataaaaatacatgcttactcctgtacaaacatcgaacaatgtaattaaatcatcactacttgaaatacttttacatgaataatttatctctttacactgttgaagccttgcatttcagtatgttctacagcttctgtatcatcacctgaaatttgcaagcaggcattgaagacacttcagctgttacaatactttttattcccaagtttgataagccacctctgattaagccacacgtaaatgctaaatacttagatgcatgttctaaatactgttttcctgcagacatctgagtaagcaggcgaaatttgttgtcctgaagtacatagatgccctgatgatttgtccttagattgtcgatttgtttcttgaataccgtagtccaaaaatctttacaaatgaacttcatgatatctaactcatccttgaaccttgcagtatcttttgtaaacctttctatcaatccttgtcccactcgaaaccccatgttttccagcttagtaatacatcgtccgttttcctgtagtcccagctactcaagaggctgaggcaggagaaacgcttgaacccaggaggcagagattgcagcgagccgagatcatgccactgcactccagtctgggtgacagggcgagacacctccccctgctccgcggacttgtacactccagacaccatctcgttatggagaagcaaaaacaacgcctcatccgccatttcctgctaattcttccaagcttcgagttttggctcccgtttgagctggtctgggggttccagctcgcgcctcagcgacttcgccggcgccgcggctccgtcaggccgccattctatccctgtggctaagagaccgaggtattcacacgacttcccaaaggctggtactgaaatgagtctggtactggagagagcccacacttcggggctaccaaatcctagggccgaactaaagtctg

SEQ ID NO: 16252 - RNA, 1500 nt, Homo sapiens
  source 1..1500: mol_type = other RNA
ggccagccaccaggagggctgcccatacaggggtgtgcggtaagaggctgcctctgttcctggtctccggtcccccttctccggcctggggttcgaggcctcgcagtatggtgtgtgttccggcagtgcctcgctcctcttgggcgccaaacccttcacgctcacctgcagctggctggtgtacttttcatgcttgagtgcctcctccgggactcggtgctgcacacgctccagcacatacatgttggaatcgtagccgaagcggatgacatcgttgagcttcagcgtgacgtacttctggtccgggatgcgcatgtcattcacaaacgtcccattgaggctgcccaggtccttcacccagtgctcgtccctgtcctggtcgtagttgatgacggcatgctgcttgtccacgctgcgggactcccaaaggccccatctcttgaagctaccacgctggaaatgaagcttcaacctccgaattgcaggggacacaaaccttcccgccacagcaggacacatgcagcaatatcgggtggggctgccctgggtagaggcagacaaacactgtctgccccagggaatgtgcacatggccaggacccctcaccacagcctgaggcctgcccacctcgtcagagcctggcatggcccgggcatgtgcggcagtagcacgttgcatccaggaggcaacgtctgagtgggcagggcagctccctgcacctgcaggcccctcggctagactggacagtgccatccacctgggtcaggggcccacgtgccacgctgggggatgagccaggacagggagcccaactcgttcacaggcacacggggtagaggaaggacatcaggccaggatgggcctatggggttagctcaccacccctgctctttgttctcaaacagccagatcgcaagccccacaaagccaaactcagacctcaaaccagggccagagaaacttccgattgtcagtgccggtgctcggcaggctctcatgccctgagaagaacccctcatgcctggaggccgccaaaaggcactagccttcaccagggtgcagctgggaccaagatactgggacccccgctcaggcagcactcacagcatagacggggcccccagacaacaagaatatggacagaccggctttccaggaccttccaaagcccagcctcagctccctctctgcaaaaggacgccaactcacgcttctagggaccccaacaactttgagaacctgacaaaagcctaagccccctcctgtcagagacagggatacgtacggggcagggacccgagcctgtgagcacacacacacccctgcacgcacccacgggagccccagagccctcggtgcatccgggacccaagttaagaggcccagcctgggctgcatggcggcctcctcgccagggtggcctgcagcaagtggggtgggcaccttcctggcctccacagggacagactgtctaccccctaccctcctggccccaagcgc

SEQ ID NO: 16253 - RNA, 1505 nt, Homo sapiens
  source 1..1505: mol_type = other RNA
ggccagccaccaggagggctgcccatacaggggtgtgcggtaagaggctgcctctgttcctggtctccggtcccccttctccggcctggggttcgaggcctcgcagtatggtgtgtgttccggcagtgcctcgctcctcttgggcgccaaacccttcacgctcacctgcagctggctggtgtacttttcatgcttgagtgcctcctccgggactcggtgctgcacacgctccagcacatacatgttggaatcgtagccgaagcggatgacatcgttgagcttcagcgtgacgtacttctggtccgggatgcgcatgtcattcacaaacgtcccattgaggctgcccaggtccttcacccagtgctcgtccctgtcctggtcgtagttgatgacggcatgctgcttgtccacgctgcgggactcccaaaggccccatctcttgaagctaccacgctggaaatgaagcttcaacctccgaattgcaggggacacaaaccttcccgccacagcaggacacatgcagcaatatcgggtggggctgccctgggtagaggcagacaaacactgtctgccccagggaatgtgcacatggccaggacccctcaccacagcctgaggcctgcccacctcgtcagagcctggcatggcccgggcatgtgcggcagtagcacgttgcatccaggaggcaacgtctgagtgggcagggcagctccctgcacctgcaggcccctcggctagactggacagtgccatccacctgggtcaggggcccacgtgccacgctgggggatgagccaggacagggagcccaactcgttcacaggcacacggggtagaggaaggacatcaggccaggatgggcctatggggttagctcaccacccctgctctttgttctcaaacagccagatcgcaagccccacaaagccaaactcagacctcaaaccagggccagagaaacttccgattgtcagtgccggtgctcggcaggctctcatgccctgagaagaacccctcatgcctggaggccgccaaaaggcactagccttcaccagggtgcagctgggaccaagatactgggacccccgctcaggcagcactcacagcatagacggggcccccagacaacaagaatatggacagaccggctttccaggaccttccaaagcccagcctcagctccctctctgcaaaaggacgccaactcacgcttctagggaccccaacaactttgagaacctgacaaaagcctaagccccctcctgtcagagacagggatacgtacggggcagggacccgagcctgtgagcacacacacacccctgcacgcacccacgggagccccagagccctcggtgcatccgggacccaagttaagaggcccagcctgggctgcatggcggcctcctcgccagggtggcctgcagcaagtggggtgggcaccttcctggcctccacagggacagactgtctaccccctaccctcctggccccaagcgctccct

SEQ ID NO: 16254 - RNA, 666 nt, Homo sapiens
  source 1..666: mol_type = other RNA
ggccagccaccaggagggctgcccatacaggggtgtgcggtaagaggctgcctctgttcctggtctccggtcccccttctccggcctggggttcgaggcctcgcagtatggtgtgtgttccggcagtgcctcgctcctcttgggcgccaaacccttcacgctcacctgcagctggctggtgtacttttcatgcttgagtgcctcctccgggactcggtgctgcacacgctccagcacatacatgttggaatcgtagccgaagcggatgacatcgttgagcttcagcgtgacgtacttctggtccgggatgcgcatgtcattcacaaacgtcccattgaggctgcccaggtccttcacccagtgctcgtccctgtcctggtcgtagttgatgacggcatgctgcttgtccacgctgcgggactgctgttcgggctcggtctccggctcgccttagtccccggcttggtccccggcttggtccccggcttgttccccagctcggcccggctcggtccctgccctcgcgcccgcccgcccgcccggccgagcgctgggcggggccgccgcctaggacatgcccggcgaggcccgcacgctcgtggcagcccgggccgagcccacggcagagcggccgccggcggcctcgcgcgcgggtccctgacgtct

SEQ ID NO: 16255 - RNA, 736 nt, Homo sapiens
  source 1..736: mol_type = other RNA
ggccagccaccaggagggctgcccatacaggggtgtgcggtaagaggctgcctctgttcctggtctccggtcccccttctccggcctggggttcgaggcctcgcagtatggtgtgtgttccggcagtgcctcgctcctcttgggcgccaaacccttcacgctcacctgcagctggctggtgtacttttcatgcttgagtgcctcctccgggactcggtgctgcacacgctccagcacatacatgttggaatcgtagccgaagcggatgacatcgttgagcttcagcgtgacgtacttctggtccgggatgcgcatgtcattcacaaacgtcccattgaggctgcccaggtccttcacccagtgctcgtccctgtcctggtcgtagttgatgacggcatgctgcttgtccacgctgcgggactgtagcatgagctcacactcctcacgccccacgaagatgagctcccgagggagccggtggcgggcgccgctgctgctcaccaggaaccaggacgtggcactcatcttggtgctggctgggcccgtctggccctgctgttcgggctcggtctccggctcgccttagtccccggcttggtccccggcttggtccccggcttgttccccagctcggcccggctcggtccctgccctcgcgcccgcccgcccgcccggccgagcgctgggcggggccgccgcctaggacatgcccggcgaggcccgcacgctcgtggca

SEQ ID NO: 16256 - RNA, 798 nt, Homo sapiens
  source 1..798: mol_type = other RNA
ggccagccaccaggagggctgcccatacaggggtgtgcggtaagaggctgcctctgttcctggtctccggtcccccttctccggcctggggttcgaggcctcgcagtatggtgtgtgttccggcagtgcctcgctcctcttgggcgccaaacccttcacgctcacctgcagctggctggtgtacttttcatgcttgagtgcctcctccgggactcggtgctgcacacgctccagcacatacatgttggaatcgtagccgaagcggatgacatcgttgagcttcagcgtgacgtacttctggtccgggatgcgcatgtcattcacaaacgtcccattgaggctgcccaggtccttcacccagtgctcgtccctgtcctggtcgtagttgatgacggcatgctgcttgtccacgctgcgggactgtagcatgagctcacactcctcacgccccacgaagatgagctcccgagggagccggtggcgggcgccgctgctgctcaccaggaaccaggacgtggcactcatcttggtgctggctgggcccgtctggccctgctgttcgggctcggtctccggctcgccttagtccccggcttggtccccggcttggtccccggcttgttccccagctcggcccggctcggtccctgccctcgcgcccgcccgcccgcccggccgagcgctgggcggggccgccgcctaggacatgcccggcgaggcccgcacgctcgtggcagcccgggccgagcccacggcagagcggccgccggcggcctcgcgcgcgggtccctgacgtct

SEQ ID NO: 16257 - RNA, 888 nt, Homo sapiens
  source 1..888: mol_type = other RNA
ggccagccaccaggagggctgcccatacaggggtgtgcggtaagaggctgcctctgttcctggtctccggtcccccttctccggcctggggttcgaggcctcgcagtatggtgtgtgttccggcagtgcctcgctcctcttgggcgccaaacccttcacgctcacctgcagctggctggtgtacttttcatgcttgagtgcctcctccgggactcggtgctgcacacgctccagcacatacatgttggaatcgtagccgaagcggatgacatcgttgagcttcagcgtgacgtacttctggtccgggatgcgcatgtcattcacaaacgtcccattgaggctgcccaggtccttcacccagtgctcgtccctgtcctggtcgtagttgatgacggcatgctgcttgtccacgctgcgggactgtagcatgagctcacactcctcacgccccacgaagatgagctcccgagggagccggtggcgggcgccgctgctgctcaccaggaaccaggacgtggcactcatcttggtgctggctgggcccgtctggccctgtgaggccggccccagagctcctgagtggacatggggctgtgactcaggaggccagtcaagaagtgaggacaataacccaggacagggatgacagcagctgaggcccagtggagcagaggagaaggggaggctgccgggctgagtgcatcctgctgttcgggctcggtctccggctcgccttagtccccggcttggtccccggcttggtccccggcttgttccccagctcggcccggctcggtccctgccctcgcgcccgcccgcccgcccggccgagcgctgggcggggccgccgcctaggacatgcccggcgaggcccgcacgctcgtggca

SEQ ID NO: 16258 - RNA, 1251 nt, Homo sapiens
  source 1..1251: mol_type = other RNA
ggccagccaccaggagggctgcccatacaggggtgtgcggtaagaggctgcctctgttcctggtctccggtcccccttctccggcctggggttcgaggcctcgcagtatggtgtgtgttccggcagtgcctcgctcctcttgggcgccaaacccttcacgctcacctgcagctggctggtgtacttttcatgcttgagtgcctcctccgggactcggtgctgcacacgctccagcacatacatgttggaatcgtagccgaagcggatgacatcgttgagcttcagcgtgacgtacttctggtccgggatgcgcatgtcattcacaaacgtcccattgaggctgcccaggtccttcacccagtgctcgtccctgtcctggtcgtagttgatgacggcatgctgcttgtccacgctgcgggactgtagcatgagctcacactcctcacgccccacgaagatgagctcccgagggagccggtggcgggcgccgctgctgctcaccaggaaccaggacgtggcactcatcttggtgctggctgggcccgtctggcccttgggcagggaggtgggaagatgtagaaaaatcctcaccaggagaaggcagctccaggcagccaggaccctctcactctgggggccctgcccttcctaagccacgcacccagctccagccagacaggcaggcactggaggccaaggggctggcacttcgatgaccctgcagccccagacagcaaagcctccaggaggcctctacagccccaccctccctagggctgctgggggagaccacagggtgctctatcgggcagggcctaccccaccattgcacctccggcccccagccagccctcctaggcctcaccctctgccatcacctgccgcggcccgccctgaggagtccacggtccctgtttaaggcgaaatgaagccgagccccagagcctggtggtgccgctgtgccagagccaggccacccactgccccggccgcccaccctgaaaaggcctgggagcccgcgacgctccaaaacggccttcggctgcctcggggctgggctggccatcgttgctaggaggaagaataataaacgccccaaacttgtcccctcagccgccccggccggaagggccacagtcagaggtgaggcggggaaaggtggctaggcccagggcagggaagggcagcgagccgggcggggcaggccggcggtggaaggagcgcacaggccgggagaggcagggacagcgg

SEQ ID NO: 16259 - RNA, 1012 nt, Homo sapiens
  source 1..1012: mol_type = other RNA
ggccccgggccctcgaccggaccggtgcgcgggcgctgcggccgcacggcgcgactgtccccgggccgggcaccgcggtccgcctctcgctcgccgcccggacgtcggggccgccccgcggggcgggcggagcgccgtccccgcctcgccgccgcccgcgggcgccggccgcgcgcgcgcgcgcgtggccgccggtccctcccggccgccgggcgcgggtcgggccgtccgcctcctcgcgggcgggcgcgacgaagaagcgtcgcgggtctgtggcgcggggccccggtggtcgtgtcgcgtggggggcgggtggttggggcgtccggttcgccgcgccccgccccggccccaccggtcccggccgccgcccccgcgcccgctcgctccctcccgtccgcccgtccgcggcccgtccgtccgtccgtcgtcctcctcgcttgcggggcgccgggcccgtcctcgcgaggccccccggccggccgtccggccgcgtcggggcctcgccgcgctctaccttacctacctggttgatcggttctcggcggcgtcgcggcgggtctgggggggtctcggtgccctcctccccgccggggcccgtcgtccggccccgccgcgccggctccccgtcttcggggccggccggattcccgtcgcctccgccgcgccgctccgcgccgccgggcacggccccgctcgctctccccggccttcccgctagggcgtctcgagggtcgggggccggacgccggtcccctcccccgcctcctcgtccgcccccccgccgtccaggtacccggcggccgtcgcgcgcctgccgcgcgtgtggcgtgcgccccgcgccgtgggggcgggaacccccgggcgcctgtggggtggtgtccgcgctcgcccccgcgtgggcggcgcgcgcctccccgtggtgtgaaaccttccgacccctctccggagtccggtcccgtttgctgtctcgtctggccggcctgaggcaaccccctctcctattgatcat

SEQ ID NO: 16260 - RNA, 2340 nt, Homo sapiens
  source 1..2340: mol_type = other RNA
ggccttgttcctgtccccatcctgtagggtcctttgagacccagccttggggaaagtgtggtcagtggggacttggcccaggccaggctctgtctggtcaccggcagaaacgcgaggaggaatcaagttcacatggggcaggaaagggcccccagacccagacaatagggcccagcaggcagggcccgagcaggtgaggagggagtagtgggctgccaggcctccctcatacccctggagctgtcctccagagccagatcagtcatctgctgagcatcaaccaggaagagttcctatccatgggaggctccatcccaacaggtgtgaagaggatgagatcttcagggagtcacccagcgggctagaaaaccaccggagtctgaccgctaagtcactgtggccagaatccaaggtcacccgaggtccaaagagaagtccaggccaggagtcctggagatgcggcccagatggagccacccccttgccgagactgtaataaagcgtgttctgacatgaagatctgagcagatgggatcatgtctctgggttcacctctgcgtccccagcatctggctcagagaagttgcttggtccatgccggtgctggcagcatccagccgacacacaggcagcccaggctcccagctccttccttccccacacagaccccacaggcccatcctggaagacaaaagagccaaccacaccgcaggagaaaactgcacccaggccccctccccaggcccaggccttgccagaactccctgctgaagaaagaaggaccaggagccagggaggctgggcccaggcaccccaccctccacctctctttattccaccccagaacatccttaaaaggtgaggggagaagggttcccaggttcccttcactcactccctgtttcccaacaacagcagaatgtgacccaggagaaagtaggacaaactcagcagcttggtgatagctgaatagcagctgaacggagagtcaggaatccagaattctgatcccagctctgctcctgccacactgggtggccctggaacccttcctgccttgacattcactcaaggtgcacggtaatcacccattgtttgaagcaatggatgggaaatggaagggacccttctgcccagcctcagttatttttctgctccccctccttctcccctgccctttcctgatgccccatgcaccagaggaaattcggggagccagaggctggactaggactcttttaagaccaccctgtgtcaccagtctggagaagaccagagaatgaccactaatcctgacctaggaccatctgccaggttttgtttttggtaacaactgtgctgtcttcatcaactggcagacctgagtcaggagagtcagggagctctctcagcatatcttcagagcttgctgtcagcacccgggagtgggggcacgagtccagaactggagatgagctcagacacttacactgagaaaaatgcatctaaagtcacagtgttaactcttcacttaactctaaggccaaggagccctgtccaaggtttataaatatgatcacaaagtgctgaaactgagaagagaagggctggttcacatcatcagggagtccccagcctccttctaatagcagttctacaagtacacaagatgaagtcatttaactcagccttcaaaagttccagacggtaatgtttgtgaaatactagccctaacgccaaatgtgaagtgtgaaaatcaccctttctgggaccccacaaaatggggacaggctctttctttcttccatagaggtagaaaagagaatgagctacatcacccatttcccctcccactttggcattctaggatactacactttcctgcacagaccagaagagggcaggctggtaggctatgggctggtaagtttaaatacttatctgcaaagatgcttctcagtgtggttgtgaacgtcctgaagaacctggaaattcccttctgtctcctctgtcccaggaacttgctgctctctgtaaatagaccctggactgctcagaggagcctggcttgatccacagtgaccctttcccctcgttctgtggaccttggttacccctgtgatgccgacggggtcatggtggccacatgaacgtgtctggaaccacatgggtggacagatgcctccaactcgggtccgcggtcctgcggcgctagtgcagagggctctttgtgccccggctcacagcgcagaactgggggagcccctgcaagcgcctcccatctcaaactcctccccgcactcgtccgcagcctccctccctctggtcccgcgagcgcagccggcgtcgtctttgtagctg

SEQ ID NO: 16261 - RNA, 2266 nt, Homo sapiens
  source 1..2266: mol_type = other RNA
ggccttgttcctgtccccatcctgtagggtcctttgagacccagccttggggaaagtgtggtcagtggggacttggcccaggccaggctctgtctggtcaccggcagaaacgcgaggaggaatcaagttcacatggggcaggaaagggcccccagacccagacaatagggcccagcaggcagggcccgagcaggtgaggagggagtagtgggctgccaggcctccctcatacccctggagctgtcctccagagccagatcagtcatctgctgagcatcaaccaggaagagttcctatccatgggaggctccatcccaacaggtgtgaagaggatgagatcttcagggagtcacccagcgggctagaaaaccaccggagtctgaccgctaagtcactgtggccagaatccaaggtcacccgaggtccaaagagaagtccaggccaggagtcctggagatgcggcccagatggagccacccccttgccgagactgtaataaagcgtgttctgacatgaagatctgagcagatgggatcatgtctctgggttcacctctgcgtccccagcatctggctcagagaagttgcttggtccatgccggtgctggcagcatccagccgacacacaggcagcccaggctcccagctccttccttccccacacagaccccacaggcccatcctggaagacaaaagagccaaccacaccgcaggagaaaactgcacccaggccccctccccaggcccaggccttgccagaactccctgctgaagaaagaaggaccaggagccagggaggctgggcccaggcaccccaccctccacctctctttattccaccccagaacatccttaaaaggtgaggggagaagggttcccaggttcccttcactcactccctgtttcccaacaacagcagaatgtgacccaggagaaagtaggacaaactcagcagcttggtgatagctgaatagcagctgaacggagagtcaggaatccagaattctgatcccagctctgctcctgccacactgggtggccctggaacccttcctgccttgacattcactcaaggtgcacggtaatcacccattgtttgaagcaatggatgggaaatggaagggacccttctgcccagcctcagttatttttctgctccccctccttctcccctgccctttcctgatgccccatgcaccagaggaaattcggggagccagaggctggactaggactcttttaagaccaccctgtgtcaccagtctggagaagaccagagaatgaccactaatcctgacctaggaccatctgccaggttttgtttttggtaacaactgtgctgtcttcatcaactggcagacctgagtcaggagagtcagggagctctctcagcatatcttcagagcttgctgtcagcacccgggagtgggggcacgagtccagaactggagatgagctcagacacttacactgagaaaaatgcatctaaagtcacagtgttaactcttcacttaactctaaggccaaggagccctgtccaaggtttataaatatgatcacaaagtgctgaaactgagaagagaagggctggttcacatcatcagggagtccccagcctccttctaatagcagttctacaagtacacaagatgaagtcatttaactcagccttcaaaagttccagacggtaatgtttgtgaaatactagccctaacgccaaatgtgaagtgtgaaaatcaccctttctgggaccccacaaaatggggacaggctctttctttcttccatagaggtagaaaagagaatgagctacatcacccatttcccctcccactttggcattctaggatactacactttcctgcacagaccagaagagggcaggctggtaggctatgggctggtaagtttaaatacttatctgcaaagatgcttctcagtgtggttgtgaacgtcctgaagaacctggaaattcccttctgtctcctctgtcccaggaacttgctgctctcttggttacccctgtgatgccgacggggtcatggtggccacatgaacgtgtctggaaccacatgggtggacagatgcctccaactcgggtccgcggtcctgcggcgctagtgcagagggctctttgtgccccggctcacagcgcagaactgggggagcccctgcaagcgcctcccatctcaaactcctccccgcactcgtccgcagcctccctccctctggtcccgcgagcgcagccggcgtcgtctttgtagctg

SEQ ID NO: 16262 - RNA, 2214 nt, Homo sapiens
  source 1..2214: mol_type = other RNA
ggccttgttcctgtccccatcctgtagggtcctttgagacccagccttggggaaagtgtggtcagtggggacttggcccaggccaggctctgtctggtcaccggcagaaacgcgaggaggaatcaagttcacatggggcaggaaagggcccccagacccagacaatagggcccagcaggcagggcccgagcaggtgaggagggagtagtgggctgccaggcctccctcatacccctggagctgtcctccagagccagatcagtcatctgctgagcatcaaccaggaagagttcctatccatgggaggctccatcccaacaggtgtgaagaggatgagatcttcagggagtcacccagcgggctagaaaaccaccggagtctgaccgctaagtcactgtggccagaatccaaggtcacccgaggtccaaagagaagtccaggccaggagtcctggagatgcggcccagatggagccacctggcagcatccagccgacacacaggcagcccaggctcccagctccttccttccccacacagaccccacaggcccatcctggaagacaaaagagccaaccacaccgcaggagaaaactgcacccaggccccctccccaggcccaggccttgccagaactccctgctgaagaaagaaggaccaggagccagggaggctgggcccaggcaccccaccctccacctctctttattccaccccagaacatccttaaaaggtgaggggagaagggttcccaggttcccttcactcactccctgtttcccaacaacagcagaatgtgacccaggagaaagtaggacaaactcagcagcttggtgatagctgaatagcagctgaacggagagtcaggaatccagaattctgatcccagctctgctcctgccacactgggtggccctggaacccttcctgccttgacattcactcaaggtgcacggtaatcacccattgtttgaagcaatggatgggaaatggaagggacccttctgcccagcctcagttatttttctgctccccctccttctcccctgccctttcctgatgccccatgcaccagaggaaattcggggagccagaggctggactaggactcttttaagaccaccctgtgtcaccagtctggagaagaccagagaatgaccactaatcctgacctaggaccatctgccaggttttgtttttggtaacaactgtgctgtcttcatcaactggcagacctgagtcaggagagtcagggagctctctcagcatatcttcagagcttgctgtcagcacccgggagtgggggcacgagtccagaactggagatgagctcagacacttacactgagaaaaatgcatctaaagtcacagtgttaactcttcacttaactctaaggccaaggagccctgtccaaggtttataaatatgatcacaaagtgctgaaactgagaagagaagggctggttcacatcatcagggagtccccagcctccttctaatagcagttctacaagtacacaagatgaagtcatttaactcagccttcaaaagttccagacggtaatgtttgtgaaatactagccctaacgccaaatgtgaagtgtgaaaatcaccctttctgggaccccacaaaatggggacaggctctttctttcttccatagaggtagaaaagagaatgagctacatcacccatttcccctcccactttggcattctaggatactacactttcctgcacagaccagaagagggcaggctggtaggctatgggctggtaagtttaaatacttatctgcaaagatgcttctcagtgtggttgtgaacgtcctgaagaacctggaaattcccttctgtctcctctgtcccaggaacttgctgctctctgtaaatagaccctggactgctcagaggagcctggcttgatccacagtgaccctttcccctcgttctgtggaccttggttacccctgtgatgccgacggggtcatggtggccacatgaacgtgtctggaaccacatgggtggacagatgcctccaactcgggtccgcggtcctgcggcgctagtgcagagggctctttgtgccccggctcacagcgcagaactgggggagcccctgcaagcgcctcccatctcaaactcctccccgcactcgtccgcagcctccctccctctggtcccgcgagcgcagccggcgtcgtctttgtagctg

SEQ ID NO: 16263 - RNA, 2140 nt, Homo sapiens
  source 1..2140: mol_type = other RNA
ggccttgttcctgtccccatcctgtagggtcctttgagacccagccttggggaaagtgtggtcagtggggacttggcccaggccaggctctgtctggtcaccggcagaaacgcgaggaggaatcaagttcacatggggcaggaaagggcccccagacccagacaatagggcccagcaggcagggcccgagcaggtgaggagggagtagtgggctgccaggcctccctcatacccctggagctgtcctccagagccagatcagtcatctgctgagcatcaaccaggaagagttcctatccatgggaggctccatcccaacaggtgtgaagaggatgagatcttcagggagtcacccagcgggctagaaaaccaccggagtctgaccgctaagtcactgtggccagaatccaaggtcacccgaggtccaaagagaagtccaggccaggagtcctggagatgcggcccagatggagccacctggcagcatccagccgacacacaggcagcccaggctcccagctccttccttccccacacagaccccacaggcccatcctggaagacaaaagagccaaccacaccgcaggagaaaactgcacccaggccccctccccaggcccaggccttgccagaactccctgctgaagaaagaaggaccaggagccagggaggctgggcccaggcaccccaccctccacctctctttattccaccccagaacatccttaaaaggtgaggggagaagggttcccaggttcccttcactcactccctgtttcccaacaacagcagaatgtgacccaggagaaagtaggacaaactcagcagcttggtgatagctgaatagcagctgaacggagagtcaggaatccagaattctgatcccagctctgctcctgccacactgggtggccctggaacccttcctgccttgacattcactcaaggtgcacggtaatcacccattgtttgaagcaatggatgggaaatggaagggacccttctgcccagcctcagttatttttctgctccccctccttctcccctgccctttcctgatgccccatgcaccagaggaaattcggggagccagaggctggactaggactcttttaagaccaccctgtgtcaccagtctggagaagaccagagaatgaccactaatcctgacctaggaccatctgccaggttttgtttttggtaacaactgtgctgtcttcatcaactggcagacctgagtcaggagagtcagggagctctctcagcatatcttcagagcttgctgtcagcacccgggagtgggggcacgagtccagaactggagatgagctcagacacttacactgagaaaaatgcatctaaagtcacagtgttaactcttcacttaactctaaggccaaggagccctgtccaaggtttataaatatgatcacaaagtgctgaaactgagaagagaagggctggttcacatcatcagggagtccccagcctccttctaatagcagttctacaagtacacaagatgaagtcatttaactcagccttcaaaagttccagacggtaatgtttgtgaaatactagccctaacgccaaatgtgaagtgtgaaaatcaccctttctgggaccccacaaaatggggacaggctctttctttcttccatagaggtagaaaagagaatgagctacatcacccatttcccctcccactttggcattctaggatactacactttcctgcacagaccagaagagggcaggctggtaggctatgggctggtaagtttaaatacttatctgcaaagatgcttctcagtgtggttgtgaacgtcctgaagaacctggaaattcccttctgtctcctctgtcccaggaacttgctgctctcttggttacccctgtgatgccgacggggtcatggtggccacatgaacgtgtctggaaccacatgggtggacagatgcctccaactcgggtccgcggtcctgcggcgctagtgcagagggctctttgtgccccggctcacagcgcagaactgggggagcccctgcaagcgcctcccatctcaaactcctccccgcactcgtccgcagcctccctccctctggtcccgcgagcgcagccggcgtcgtctttgtagctg

SEQ ID NO: 16264 - RNA, 114 nt, Homo sapiens
  source 1..114: mol_type = other RNA
ggcggcggcggaggcgggggcggcggctgaggcgggaagcagccggccaggcccgggcgccgcgggctggctctggccaagcgtcggtctccaccggcggcggcgctcgccagc

SEQ ID NO: 16265 - RNA, 4687 nt, Homo sapiens
  source 1..4687: mol_type = other RNA
ggcggcggcggaggcgggggcggcggggagcggcccggctgtgagcgcccggatgctggacgtgggggcccgaccacctcagccgcgtacgagtcctcggtgcagactgactgcagtttgctgaggatgctgcggtggccgcggcggccctggcccaggaggtagtagccggagtagacgggcggcgactcgcactgcatgcggtcgtacgtctgtgtggcgttggtgaaggcggccagccagcgcaggaagcccagcagctcgcaggagcagtagaaggggttgctgtagagctcgcacaccgacagcttggccaggccggcgaaggtgccgctgttgagctgctggatgcggttcatggacaggtcgatgttgacgatgttgggacactcccagaagctgctggccatgaccacctcgatgaggttggcctgcaggtacaggtactccagcttgcccaggccgcgcagcatgccctccgtgaggttgcgcagccggttgtagcccagctgcagcacctgcaggttgaactggcccgagaaggcgccgtcctcgatgtagccgatctcgttcttggtgaggttgaggtacgtgaggttgccaaagcggctgagcgaggcgtactgcacgctgcggatacggttctcgttgagccgcaggtccacgatggtgctgttgatctgctgtgggatggcctcgtaggggggttggttctggctgcagatggccagccacacgaagcccttgtcgccctcgatcagccagcagtctgcgcgggccaggccgccagcgtgcagcagggtggcggccgccacgcacacccacagcgcgccccacccacgcccggccatcgggaccgccctgcagggagccccaattcagcctgcccagggggaccaggtggggggccaggcgccagcccccagagggatggaggggcgggagggggaggtgcctgcactctcaggggtgtcctgtcccaaaccgcatggccgcgcgacgtaagcgcggggagggagggcgcctccctcacggccggccgcctctcgtcttccgccccagtcctgtggtgaccgaggcctcctgccccatgggcctgggtgtcctgatggctccactgactcctcctgctccgacgttcctgctggcaggaaagacatccttcatcattctcccttttctgcgtttctttagtcttgccatttgaatattcattcagatgaacttttagaatgattttatctcgctttgtaaaactcgctgcgagcctgttgatggatggtggtaaacctgtgaattaattctggaaagactttcgggtaatattccaacacggcacatctcaccactcttgttttctttgatatctctcaggataactttagagagtttttcataatgatcctaaatttctcttgtcgattcattcctgggaattgggagggttttgttgttttattggtgccgttgtaagtggggaccgtttatttaattatgtgtctcgactagctgttgttagttcagagaaaagttattgatttgtatatgttggtttgatttccagcccagcaccttcgtattaaatttttatattaagtcattttttttctcagttgcttctcttgggtttctaagatcttgaatcattttgtcagcaaataattacaattcttccctgtagacatcccatttaattctgtttcatgtcttattgctatgtccagaatttctggacaatgatgaaagcattgctgttttttaatataagtttctgaatgggaatcattaaaaaatctcatcacctagaatgattctggctgttgaactgagacagattcttgacttcgataaagacgtgtgtttctggttctatttctagcagttactttaaaatccgaaattggcactggattttatcaaatgcctttcgtcattatgaatgtgcattccagctgacctgtggacactgtgtagtttattaatagatttatctaatattaagccaactttgaattttttgtataacttctacataatcatggccgattcttatctctgtgatattctgtggaattggatttccttgagtgtctttgaggctttttgatccaatattcacgggtgagatcagggtggggtttcatttcctgcagggtcttggctggtttggggtttgaggctgtcctggcttcctcctccagctcatcaaacagtgttgctgctggaagcccctggctctgtaggcttggcccccctccccagtggatgtgttccggaaagtcctgcaggcaaacaccacacactgctttgtaaagtgaatgatcattttctcaagtgaaatgtcacgcctcatttgtcttctgtgctttccagattttcacgattcagggtcagctcaaagcagggtgaacgatagagaagcctcctctgggagagctcatgaccgcctggaaggcatccgacgtggcggattcggagatggcatctgggaggggctggtccccgggtggggctgccgagggccttggagggtgaccccagctccctgcccttgaggctaggcctgtgagaccacccccgcccacctcctggggcctgctggtctacgtgcctcggcatccgtgctgacagatggacatcccagtaggcatttgagaggggagggcacagacaatacaaaatgaataaactgcaatctcagccccttcgggacggctgttctaacataggagaaaaggaacagacgcaggaagtaaataggggctcaaggcaggactactagggccgaccctgtctgcaaaagacagctgcgtctctacctcccacctggagtctgcagagaccttgacaccccctgctgagacacagggtctagctcagcacgcctgaatctgggctggcctgagacagccttaaccaaggcgctggtagaagcgaagccgtgtccgtcctgggcacagcccctagctaggccggccaccctgcctcctgtgtcctagaagcagccaccaggtgagaaaagcgactttcccagcaccctgctgtgaggcctgggtggtggggggtgtggtcccatcgagactgagaggctagggccatggcactggcttgggagtgaaggagccgctgctgagcagaggtgaaccgccctgctgagcccttcccagtgcctgacccaagaaccctgagcaaaagaagctggccctgagccccggggtgcaggactttgtgggacagtggaggatcactgactcacaccaaacccaagtcctcaagtaagagggagtgggtggggagccccaggcctcctccaagctcacgttccccatccaccacagggggccaagctctggctctaagaatccactggagaattggagggctcctggcagtgagttgagcagaggggccctgtgtggtgtgagggccagaggaagctggcagtggcagctccgcggggcaggaggagctgggctttaagctgagtttgcctcctgagcagccggctgctccccagctgggtgatttgcagaatgtccttaagttctttgagcctcagtttacctttctgacaaatggggccactgatagccatcatgagatgatggacatcatgagatgatgaacaggaccatcacgacagtgagatgcgatggtgtttgtgaacacgctggacacacggaggagctggtgtgaaactccccttccccgacaggagctgggacccgggtggagctggatcctcccactcagttcctgatactcacaaaactctgggtctttcccagcctctgttttctctcctctgaaaactgaaaatactaacatcaccctggggttcctggaggggggaacgtgagaaaacgcatgtgctgtgtgctgcctggggcgtgaagtggtccaaaagccatcggtgggatttgcatggacagaaggaaaggtggggggtctgagcaaagcccaggaggtgcctccgaaccaggggaccctgagcgctggggcagtggctttctgtgagggaaggtggccaggaccctgagtgaagaggactgggtgcctgttggcagcagctggcttctgctcgcccagccagctctgcaaaccctccgcatctcagagcctatcaagaatctctctaataacacagcaaacattaattacagctgaaaggccgcagaatgcggttggtctgaaagaggctgccccttgttagtcagtgagcctctgggaagggtgcaggccggggctgggctccctccacaggggctactgcagtggcagggggatggggagcaggagtcactcccagggctacagtgcagaccacaggtcctgggggagaccttctgttctcacccgtttggcgccctaagggaaagcctgtcctcgcaacctggagcaggagaggcaaaaagagaggcccctgggtggagcaggaaggtctgggatccaagtccggccctgcctctcaatggctctggacagaaaaccgcccatgcaaaggggtggtgcttggacctctcggcctctctcaaaccgctcccctgcacacagggtggagagaaggcccattccctgggcattcaaaagtccaacaggctgcaaataaggactaggggaggtgaggcacagtggctcacccctgtaatcctggagctttgggagggcaaggtgggaggattgcttg

SEQ ID NO: 16266 - RNA, 1585 nt, Homo sapiens
  source 1..1585: mol_type = other RNA
ggcggcggcggaggcgggggcggcggggagcggcccggctgtgagcgcccggatgctggacgtgggggcccgaccacctcagccgcgtacgagtcctcggtgcagactgactgcagtttgctgaggatgctgcggtggccgcggcggccctggcccaggaggtagtagccggagtagacgggcggcgactcgcactgcatgcggtcgtacgtctgtgtggcgttggtgaaggcggccagccagcgcaggaagcccagcagctcgcaggagcagtagaaggggttgctgtagagctcgcacaccgacagcttggccaggccggcgaaggtgccgctgttgagctgctggatgcggttcatggacaggtcgatgttgacgatgttgggacactcccagaagctgctggccatgaccacctcgatgaggttggcctgcaggtacaggtactccagcttgcccaggccgcgcagcatgccctccgtgaggttgcgcagccggttgtagcccagctgcagcacctgcaggttgaactggcccgagaaggcgccgtcctcgatgtagccgatctcgttcttggtgaggttgaggtacgtgaggttgccaaagcggctgagcgaggcgtactgcacgctgcggatacggttctcgttgagccgcaggtccacgatggtgctgttgatctgctgtgggatggcctcgtaggggggttggttctggctgcagatggccagccacacgaagcccttgtcgccctcgatcagccagcagtctgcgcgggccaggccgccagcgtgcagcagggtggcggccgccacgcacacccacagcgcgccccacccacgcccggccatcgggaccgccctgcagggagccccaattcagcctgcccagggggaccaggtggggggccaggcgccagcccccagagggatggaggggcgggagggggaggtgcctgcactctcaggggtgtcctgtcccaaaccgcatggccgcgcgacgtaagcgcggggagggagggcgcctccctcacggccggccgcctctcgtcttccgccccagtcctgtggtgaccgaggcctcctgccccatgggcctgggtgtcctgatggctccactgactcctcctgctccgacgttcctgttgtgtgtcagggcccgccaacgacctgatgcaccagcgaggaataggctggaggattcctccctgctgggctcaaagacatgttcgcctcattccagcacacagaaggacagcctgggtccggacaaactgtaggacaaatggtcgccaaggcagctgcaccaggcctcaggagtgtggctctggttcaggtgcccactggcttttctgggagtcgggagctgcctgccgagcctgctgtatcatcctgaattatacgcacacagcagtcctgctgcggccgaggaggagggggctgcacagctggctgcccgcccggcctcggttccggggctgcgcccgcagccgccgccgtccttcaagctctaacttcgctcccgggattgaaattcctccccagcttcgcccatcgatctgcgcgcgcggccccgcccctcgccg

SEQ ID NO: 16267 - RNA, 2943 nt, Homo sapiens
  source 1..2943: mol_type = other RNA
ggcggcggcggaggcgggggcggcggggagcggcccggctgtgagcgcccggatgctggacgtgggggcccgaccacctcagccgcgtacgagtcctcggtgcagactgactgcagtttgctgaggatgctgcggtggccgcggcggccctggcccaggaggtagtagccggagtagacgggcggcgactcgcactgcatgcggtcgtacgtctgtgtggcgttggtgaaggcggccagccagcgcaggaagcccagcagctcgcaggagcagtagaaggggttgctgtagagctcgcacaccgacagcttggccaggccggcgaaggtgccgctgttgagctgctggatgcggttcatggacaggtcgatgttgacgatgttgggacactcccagaagctgctggccatgaccacctcgatgaggttggcctgcaggtacaggtactccagcttgcccaggccgcgcagcatgccctccgtgaggttgcgcagccggttgtagcccagctgcagcacctgcaggttgaactggcccgagaaggcgccgtcctcgatgtagccgatctcgttcttggtgaggttgaggtacgtgaggttgccaaagcggctgagcgaggcgtactgcacgctgcggatacggttctcgttgagccgcaggtccacgatggtgctgttgatctgctgtgggatggcctcgtaggggggttggttctggctgcagatggccagccacacgaagcccttgtcgccctcgatcagccagcagtctgcgcgggccaggccgccagcgtgcagcagggtggcggccgccacgcacacccacagcgcgccccacccacgcccggccatcgggaccgccctgcagggagccccaattcagcctgcccagggggaccaggtggggggccaggcgccagcccccagagggatggaggggcgggagggggaggtgcctgcactctcaggggtgtcctgtcccaaaccgcatggccgcgcgacgtaagcgcggggagggagggcgcctccctcacggccggccgcctctcgtcttccgccccagtcctgtggtgaccgaggcctcctgccccatgggcctgggtgtcctgatggctccactgactcctcctgctccgacgttcctgttgtgtgtcagggcccgccaacgacctgatgcaccagcgaggaataggctggaggattcctccctgctgggctcaaagacatgttcgcctcattccagcacacagaaggacagcctgggtccggacaaactgtaggacaaatggtcgccaaggcagctgcaccaggcctcaggagtgtggctctggttcaggtgcccactggcttttctgggagtcgggagctgcctgccgagcctgctgtatcatcctgaattatacgcacacagcagtcctgctgcggccgaggaggagggggctgcacagctggctgtaggacagggggaggggcatggcccccaatctctgacttggagacccccaggtcttctgcccactaggggtggggatcagaactccctgaccaccgtatgcccaggaaaatgagggacccaagtgctggggtcctggctgggctccaaaccccctcaaatccaggtgagggggtgaccccctcccacacacggccccctggagtttgtccccctgctttggtggagtggggcgcaaacctgggctgggacctgtaagccagtcttctcaatgcttgttcaattaaaaggtggcaggggcagggacccagggggcaggaggccagggggccagccaggcagagaagaggagcatgttgatgcttttcaagcaacctatgcccaacccaatggggtttcccccaaggctgggtgcaagctggacctctttggaggctgggggcctctctagggggcagcccctgagagaggcaatatggggagatttgccatttacatctgctcctggctcccggtccctccacagcttctgtccccaggctctccgcacagcccttagcccaatcgagggaatgagcggcagaggcagccagcccaagccagggtccaaagaggccccactccgggtgtgcaggaagggaaagtgctggcacggaggctttttgaggacgtgcacacctggctcggccggcctcgaccctttctgctaagccttcgtttttttcagaaggcatgatcatcctagccccatttcacaggtgtggaaactgaggctctgagattcacctgccccaaggtcacacagctgagacctggaaaagccggattttcatctcagagggtgtcgtttttatgggggggggggcggtgtgcggtacggcaggcagtgccccccgccccaccctcagcatcaagcaggtgacctgcaggtttcaaaggatggaaatgggggcgcttgtctttagaggcaggttggggcacggaggcttggcagcctcctcccagcccccagagggacgaggacgaggatggactccaggtggggcgaggggtggaaagcacccagtaagttcagttcggagcgaagccccccaccccacccccccgccagtggttggactcaggggctgggaccgaggaatgtgacccctccccgtgcgtgactggacggtccccgcgcggagcgaggaggctcgcagcgtcggggggagggcggcccagcagggagggcgatgcgagcctggggaggggtcagcgactcggccaggaggtgaggacagccccctaatttccgggaagggaagggcagggggccgcgtctggggggcgccgggcagggtgcggacggcgaagggggacggaagggagagaggcgctggggaagggacctctcggaggcacggggcagcgtgcgggctgcggcagcgaccccgacccgggcccccgggctttgtcgggctgagcctgcgcccgctccgccgccgccaagtt

SEQ ID NO: 16268 - RNA, 1648 nt, Homo sapiens
  source 1..1648: mol_type = other RNA
ggcggcggcggaggcgggggcggcggggagcggcccggctgtgagcgcccggatgctggacgtgggggcccgaccacctcagccgcgtacgagtcctcggtgcagactgactgcagtttgctgaggatgctgcggtggccgcggcggccctggcccaggaggtagtagccggagtagacgggcggcgactcgcactgcatgcggtcgtacgtctgtgtggcgttggtgaaggcggccagccagcgcaggaagcccagcagctcgcaggagcagtagaaggggttgctgtagagctcgcacaccgacagcttggccaggccggcgaaggtgccgctgttgagctgctggatgcggttcatggacaggtcgatgttgacgatgttgggacactcccagaagctgctggccatgaccacctcgatgaggttggcctgcaggtacaggtactccagcttgcccaggccgcgcagcatgccctccgtgaggttgcgcagccggttgtagcccagctgcagcacctgcaggttgaactggcccgagaaggcgccgtcctcgatgtagccgatctcgttcttggtgaggttgaggtacgtgaggttgccaaagcggctgagcgaggcgtactgcacgctgcggatacggttctcgttgagccgcaggtccacgatggtgctgttgatctgctgtgggatggcctcgtaggggggttggttctggctgcagatggccagccacacgaagcccttgtcgccctcgatcagccagcagtctgcgcgggccaggccgccagcgtgcagcagggtggcggccgccacgcacacccacagcgcgccccacccacgcccggccatcgggaccgccctgcagggagccccaattcagcctgcccagggggaccaggtggggggccaggcgccagcccccagagggatggaggggcgggagggggaggtgcctgcactctcaggggtgtcctgtcccaaaccgcatggccgcgcgacgtaagcgcggggagggagggcgcctccctcacggccggccgcctctcgtcttccgccccagtcctgtggtgaccgaggcctcctgccccatgggcctgggtgtcctgatggctccactgactcctcctgctccgacgttcctgttgtgtgtcagggcccgccaacgacctgatgcaccagcgaggaataggctggaggattcctccctgctgggctcaaagacatgttcgcctcattccagcacacagaaggacagcctgggtccggacaaactgtaggacaaatggtcgccaaggcagctgcacccagccctggtgctgaggattctccaggcctcatctcatttcaccagcgtacttgcttccttcaccacgaggtggcacctgatccccattttgcagatagggaaactgaggctgagaagggaagtcgtcctgccagggtcgcacagctggggtgtggtgcagagcccagccccatgaatgatgcttttgcatctggagggcaggaggggaagtgctgtggggtgctggtggggtgcagggaccagaggaggtagtgtctgcaagacaaaggggggttctaggtgcaaaggggttcgcgaggttggtgcagaggcggggggttggtgctgggctctgccgcat

SEQ ID NO: 16269 - RNA, 1440 nt, Homo sapiens
  source 1..1440: mol_type = other RNA
ggcggcggcggaggcgggggcggcggggagcggcccggctgtgagcgcccggatgctggacgtgggggcccgaccacctcagccgcgtacgagtcctcggtgcagactgactgcagtttgctgaggatgctgcggtggccgcggcggccctggcccaggaggtagtagccggagtagacgggcggcgactcgcactgcatgcggtcgtacgtctgtgtggcgttggtgaaggcggccagccagcgcaggaagcccagcagctcgcaggagcagtagaaggggttgctgtagagctcgcacaccgacagcttggccaggccggcgaaggtgccgctgttgagctgctggatgcggttcatggacaggtcgatgttgacgatgttgggacactcccagaagctgctggccatgaccacctcgatgaggttggcctgcaggtacaggtactccagcttgcccaggccgcgcagcatgccctccgtgaggttgcgcagccggttgtagcccagctgcagcacctgcaggttgaactggcccgagaaggcgccgtcctcgatgtagccgatctcgttcttggtgaggttgaggtacgtgaggttgccaaagcggctgagcgaggcgtactgcacgctgcggatacggttctcgttgagccgcaggtccacgatggtgctgttgatctgctgtgggatggcctcgtaggggggttggttctggctgcagatggccagccacacgaagcccttgtcgccctcgatcagccagcagtctgcgcgggccaggccgccagcgtgcagcagggtggcggccgccacgcacacccacagcgcgccccacccacgcccggccatcgggaccgccctgcagggagccccaattcagcctgcccagggggaccaggtggggggccaggcgccagcccccagagggatggaggggcgggagggggaggtgcctgcactctcaggggtgtcctgtcccaaaccgcatggccgcgcgacgtaagcgcggggagggagggcgcctccctcacggccggccgcctctcgtcttccgccccagtcctgtggtgaccgaggcctcctgccccatgggcctgggtgtcctgatggctccactgactcctcctgctccgacgttcctgttgtgtgtcagggcccgccaacgacctgatgcaccagcgaggaataggctggaggattcctccctgctgggctcaaagacatgttcgcctcattccagcacacagaaggacagcctgggtccggacaaactgtaggacaaatggtcgccaaggcagctgcacctgcccgcccggcctcggttccggggctgcgcccgcagccgccgccgtccttcaagctctaacttcgctcccgggattgaaattcctccccagcttcgcccatcgatctgcgcgcgcggccccgcccctcgccg

SEQ ID NO: 16270 - RNA, 1402 nt, Homo sapiens
  source 1..1402: mol_type = other RNA
ggcggcggcggaggcgggggcggcggggagcggcccggctgtgagcgcccggatgctggacgtgggggcccgaccacctcagccgcgtacgagtcctcggtgcagactgactgcagtttgctgaggatgctgcggtggccgcggcggccctggcccaggaggtagtagccggagtagacgggcggcgactcgcactgcatgcggtcgtacgtctgtgtggcgttggtgaaggcggccagccagcgcaggaagcccagcagctcgcaggagcagtagaaggggttgctgtagagctcgcacaccgacagcttggccaggccggcgaaggtgccgctgttgagctgctggatgcggttcatggacaggtcgatgttgacgatgttgggacactcccagaagctgctggccatgaccacctcgatgaggttggcctgcaggtacaggtactccagcttgcccaggccgcgcagcatgccctccgtgaggttgcgcagccggttgtagcccagctgcagcacctgcaggttgaactggcccgagaaggcgccgtcctcgatgtagccgatctcgttcttggtgaggttgaggtacgtgaggttgccaaagcggctgagcgaggcgtactgcacgctgcggatacggttctcgttgagccgcaggtccacgatggtgctgttgatctgctgtgggatggcctcgtaggggggttggttctggctgcagatggccagccacacgaagcccttgtcgccctcgatcagccagcagtctgcgcgggccaggccgccagcgtgcagcagggtggcggccgccacgcacacccacagcgcgccccacccacgcccggccatcgggaccgccctgcagggagccccaattcagcctgcccagggggaccaggtggggggccaggcgccagcccccagagggatggaggggcgggagggggaggtgcctgcactctcaggggtgtcctgtcccaaaccgcatggccgcgcgacgtaagcgcggggagggagggcgcctccctcacggccggccgcctctcgtcttccgccccagtcctgtggtgaccgaggcctcctgccccatgggcctgggtgtcctgatggctccactgactcctcctgctccgacgttcctgttgtgtgtcagggcccgccaacgacctgatgcaccagcgaggaataggctggaggattcctccctgctgggctcaaagacatgttcgcctcattccagcacacagaaggacagcctgggtccggacaaactgtaggacaaatggtcgccaaggcagctgcacctgggccggggtgcgggccccgggctggaggcactgtcgcgggcgagcagagcgcgcgcaccccggttccccgagcgcggcggcggcggcggcggc

SEQ ID NO: 16271 - RNA, 1338 nt, Homo sapiens
  source 1..1338: mol_type = other RNA
ggcggcggcggaggcgggggcggcggggagcggcccggctgtgagcgcccggatgctggacgtgggggcccgaccacctcagccgcgtacgagtcctcggtgcagactgactgcagtttgctgaggatgctgcggtggccgcggcggccctggcccaggaggtagtagccggagtagacgggcggcgactcgcactgcatgcggtcgtacgtctgtgtggcgttggtgaaggcggccagccagcgcaggaagcccagcagctcgcaggagcagtagaaggggttgctgtagagctcgcacaccgacagcttggccaggccggcgaaggtgccgctgttgagctgctggatgcggttcatggacaggtcgatgttgacgatgttgggacactcccagaagctgctggccatgaccacctcgatgaggttggcctgcaggtacaggtactccagcttgcccaggccgcgcagcatgccctccgtgaggttgcgcagccggttgtagcccagctgcagcacctgcaggttgaactggcccgagaaggcgccgtcctcgatgtagccgatctcgttcttggtgaggttgaggtacgtgaggttgccaaagcggctgagcgaggcgtactgcacgctgcggatacggttctcgttgagccgcaggtccacgatggtgctgttgatctgctgtgggatggcctcgtaggggggttggttctggctgcagatggccagccacacgaagcccttgtcgccctcgatcagccagcagtctgcgcgggccaggccgccagcgtgcagcagggtggcggccgccacgcacacccacagcgcgccccacccacgcccggccatcgggaccgccctgcagggagccccaattcagcctgcccagggggaccaggtggggggccaggcgccagcccccagagggatggaggggcgggagggggaggtgcctgcactctcaggggtgtcctgtcccaaaccgcatggccgcgcgacgtaagcgcggggagggagggcgcctccctcacggccggccgcctctcgtcttccgccccagtcctgtggtgaccgaggcctcctgccccatgggcctgggtgtcctgatggctccactgactcctcctgctccgacgttcctgttgtgtgtcagggcccgccaacgacctgatgcaccagcgaggaataggctggaggattcctccctgctgggctcaaagacatgttcgcctcattccagcacacagaaggacagcctgggtccggacaaactgtaggacaaatggtcgccaaggcagctgcacctgtaatcccagcactttgggagaccaacgta

SEQ ID NO: 16272 - RNA, 638 nt, Homo sapiens
  source 1..638: mol_type = other RNA
ggcggcggcggaggcggggggcgcggcctcggccgcgggcgccgacactggcgggggtggcggagggggcgccggaggctgcttcagggccgctgtgtccaccgtagaggcggcggcaggggccgggggcgcggcagcgacggcggcagcagcggcggcagcggccgcagcagccgcggcggactcctgggcggcggcgagcaccgggagcaagtccacctggaggggctcggccgccggggcctggggcgtgggcgggggcgccggcgcggcctggaatggactctgggcgcagccctgggaggcaaagaagcgggactggagctcagccccgacctgcagggggttctgggcgtgaccctgaggtggcgggaaggagttcatgaggccgcccaccccccgggagtccaggcccagcacggggaaggggggggccagcagcgtgcaaggaaacaccgggaacatggcctcggccgcagcggggcccccggggctcagcgggggccgggggcgcgggccgcgcggggcccgggctcggggcgccgcccccggccggccgggctgggccgcgccgaacgcatggcccgcgggccgccccgccgcccgcgcaccccggccggcgggagggaggaaaagag

SEQ ID NO: 16273 - RNA, 790 nt, Homo sapiens
  source 1..790: mol_type = other RNA
ggcggcggcggaggcggggggcgcggcctcggccgcgggcgccgacactggcgggggtggcggagggggcgccggaggctgcttcagggccgctgtgtccaccgtagaggcggcggcaggggccgggggcgcggcagcgacggcggcagcagcggcggcagcggccgcagcagccgcggcggactcctgggcggcggcgagcaccgggagcaagtccacctggaggggctcggccgccggggcctggggcgtgggcgggggcgccggcgcggcctggaatggactctgggcgcagccctgggaggcaaagaagcgggactggagctcagccccgacctgcagggggttctgggcgtgaccctgaggtggcgggaaggagttcatgaggccgcccaccccccgggagtccaggcccagcacggggaaggggggggccagcagcgtgcaaggaaacaccgggaacatggcctcggccgcagcggggcccccggggctcagcgggggccgggggcgcgggccgcgcggggcccgggctcggggcgccgcccccggccggccgggctgggccgcgccgaacgcatggcccgcgggccgccccgccgcccgcgcaccccggccggcgggagggaggaaaagagggcgccttgcgggccgcggagcgccgcggcgacggcggcggcgacgccccctgggtgggggcgggaggccccgcggggccggggccgggggcgggggcccgggcggcggcggcggcggcggcggcggttggagcctggcggggcggggtggg

SEQ ID NO: 16274 - RNA, 417 nt, Homo sapiens
  source 1..417: mol_type = other RNA
ggcggcggcggaggcggggggcgcggcctcggccgcgggcgccgacactggcgggggtggcggagggggcgccggaggctgcttcagggccgctgtgtccaccgtagaggcggcggcaggggccgggggcgcggcagcgacggcggcagcagcggcggcagcggccgcagcagccgcggcggactcctgggcggcggcgagcaccgggagcaagtccacctggaggggctcggccgccggggcctggggcgtgggcgggggcgccggcgcggcctggaatggactctgggcgcagccctgggaggcaaagaagcgggactggagctcagccccgacctgcagggggttctgggcgtgaccctggaagatgaagctgctccagttgctgggatccatggcggagggagggagggaggt

SEQ ID NO: 16275 - RNA, 460 nt, Homo sapiens
  source 1..460: mol_type = other RNA
ggcggcggcggaggcggggggcgcggcctcggccgcgggcgccgacactggcgggggtggcggagggggcgccggaggctgcttcagggccgctgtgtccaccgtagaggcggcggcaggggccgggggcgcggcagcgacggcggcagcagcggcggcagcggccgcagcagccgcggcggactcctgggcggcggcgagcaccgggagcaagtccacctggaggggctcggccgccggggcctggggcgtgggcgggggcgccggcgcggcctggaatggactctgggcgcagccctgggaggcaaagaagcgggactggagctcagccccgacctgcagggggttctgggcgtgaccctggaagatgaagctgctccagttgctgggatccatggcggagggagggagggaggtggctcgcgctcaccctggggcgggaggaggaggcggcggcggt

SEQ ID NO: 16276 - RNA, 122 nt, Homo sapiens
  source 1..122: mol_type = other RNA
ggcggcggcggaggcggggggcggctcggggcggccggcccgcctgggctcagcctgcggtcgcggcggcggcggcggcggccccgaagacgcggcgggcgggctgcggggagggcggcggc

SEQ ID NO: 16277 - RNA, 1284 nt, Homo sapiens
  source 1..1284: mol_type = other RNA
ggcggcggcggaggcgggggtgcggccggcgggcctcccaggccattgtacgagttcactacgccggggggcagcgccatgctctgcacgcgtgtgtacggcccgtacgaggcggccgggcccgccagccccttgaccacagcggccgcgccagggctaccggggcccgcggctgcagccgcagctgctgcagccgctgcggctgccgccatctggcaggaggcatagggcatgggtgagggaggctgcggtagcggccacgagttgttgaggaagccagactgcaggtacttggggggcgccaggtagccgtagccgtcggccccggcgcccgccacgccgcacccgcctgcggcgcctccggccccgaagagccccttgccgggctggaagtgcgcgggcggcggccggaagggcctcttcatgcggcggcggcgccggtagttgcccttctcgaacatgtcttcgcaggccgggtccagcgtccagtagttgcccttgcgctcgccgccgccctcgcgcggcaccttgatgaagcactcgttgaggctgaggttgtggcggatgctattttgccagcccttcttattcttctcgtagaacgggaacttcgcgatgatgtactggtagatgccggacagcgtgagcctcttctccgcgctctcgcggatcgccatggcgatgagcgccacgtacgagtacgggggcttctgcgccgggtccggcttctccggggctgtcccgccgccacccccaccgcccttgcctgggctcggcggcggcccttctggctccttgactgtgcgaccggtctctggggccagcagggcccccgccgcgtcctcgggctcggggtagctggccatcatgacaaagccggcgcgccgcggccgggccgcctctgctctccgctccaggcgctggcgcggcaaagagttggggcgcacgagtccgcttacggccaagtctcaaacttctggagactgcggatgccgcccgcgcttgcttgctggaggcctgtcgctgctctcccctctccttccccttcccctagggagcggccggcgggagtggagctcagcctctggccatggggagtccgcccaacagagaggggctccggcctcgccgcccctccccgctcaggccagtccccgccttggtgggttttcttttctgcgctcttcccctccccccgccccccggtttcccgaagcacgacccgcgtctctggcggagctgcctcctggagtccctagtgcgccaggagcctcgctctgttct

SEQ ID NO: 16278 - RNA, 22 nt, Homo sapiens
  source 1..22: mol_type = other RNA
ggcggggctcggagccgggatt

SEQ ID NO: 16279 - RNA, 76 nt, Homo sapiens
  source 1..76: mol_type = other RNA
ggcggggctcggagccgggattccaggccggtcagctggaggcgggccgcaccactcggcctgcggagacggggag

SEQ ID NO: 16280 - RNA, 455 nt, Homo sapiens
  source 1..455: mol_type = other RNA
ggcggggctcggagccgggcgcctcggggaaggcgggcagcgggggcggcggcgcgggccccggcccgggggcggagaaggcgaaggcgcagggcgtctcggcggcggcggcgggggcgcgacggaaggcggctgagtgcaggcgcagagccgggtgcgcgtcgagcacgagcgcgcggggcgcgggccgcagcgcgcacagctcgagcaccaggcagccggccaactcgcgcgcctcgggccgcagctccaggcccagctgcaggtggcggaggcggaagagctgcgcgctggaggccgaggccacgtccagggcgggcggcggctcgggcggcgggcggacgggcgcggcctcggcgccgggcgcctggcggcagcagcactgcgcggccatggccgccggcactaggtgaaatccatgggcggcggccgcgccgggccgcgggcgaggggcg

SEQ ID NO: 16281 - RNA, 497 nt, Homo sapiens
  source 1..497: mol_type = other RNA
ggcggggctcggagccgggcgcctcggggaaggcgggcagcgggggcggcggcgcgggccccggcccgggggcggagaaggcgaaggcgcagggcgtctcggcggcggcggcgggggcgcgacggaaggcggctgagtgcaggcgcagagccgggtgcgcgtcgagcacgagcgcgcggggcgcgggccgcagcgcgcacagctcgagcaccaggcagccggccaactcgcgcgcctcgggccgcagctccaggcccagctgcaggtggcggaggcggaagagctgcgcgctggaggccgaggccacgtccagggcgggcggcggctcgggcggcgggcggacgggcgcggcctcggcgccgggcgcctggcggcagcagcactgcgcggccatggccgccggcactaggtgaaatccatgggcggcggccgcgccgggccgcgggcgaggggcgccgggcggcggcggcggcggggcgcgggcacaacaggaagtc

SEQ ID NO: 16282 - RNA, 1040 nt, Homo sapiens
  source 1..1040: mol_type = other RNA
ggcggggctcggagccgggcttcggccgggccccgggccctcgaccggaccggtgcgcgggcgctgcggccgcacggcgcgactgtccccgggccgggcaccgcggtccgcctctcgctcgccgcccggacgtcggggccgccccgcggggcgggcggagcgccgtccccgcctcgccgccgcccgcgggcgccggccgcgcgcgcgcgcgcgtggccgccggtccctcccggccgccgggcgcgggtcgggccgtccgcctcctcgcgggcgggcgcgacgaagaagcgtcgcgggtctgtggcgcggggccccggtggtcgtgtcgcgtggggggcgggtggttggggcgtccggttcgccgcgccccgccccggccccaccggtcccggccgccgcccccgcgcccgctcgctccctcccgtccgcccgtccgcggcccgtccgtccgtccgtcgtcctcctcgcttgcggggcgccgggcccgtcctcgcgaggccccccggccggccgtccggccgcgtcggggcctcgccgcgctctaccttacctacctggttgatcggttctcggcggcgtcgcggcgggtctgggggggtctcggtgccctcctccccgccggggcccgtcgtccggccccgccgcgccggctccccgtcttcggggccggccggattcccgtcgcctccgccgcgccgctccgcgccgccgggcacggccccgctcgctctccccggccttcccgctagggcgtctcgagggtcgggggccggacgccggtcccctcccccgcctcctcgtccgcccccccgccgtccaggtacccggcggccgtcgcgcgcctgccgcgcgtgtggcgtgcgccccgcgccgtgggggcgggaacccccgggcgcctgtggggtggtgtccgcgctcgcccccgcgtgggcggcgcgcgcctccccgtggtgtgaaaccttccgacccctctccggagtccggtcccgtttgctgtctcgtctggccggcctgaggcaaccccctctcctattgatcat

SEQ ID NO: 16283 - RNA, 2165 nt, Homo sapiens
  source 1..2165: mol_type = other RNA
ggctcaatctctggtcctgcagcctgacactcattggctggtatctgggctaaatctttctcctacccccacccccacttgaactcactccctgggccctggagccactctgctgaccactggcccagaagaagtcccatggcagaaacagaggcctgtgctctctctctggggctcctcagccctctccagtggctctaaagcagccccatccagtagaactttgagccgcggtcggaatggtttacatgggctcatccaatagggcagccacgagccgtgtctgtggagcatttggatgcggctagcacaaccaagtaactgaacatttaactttatttgattttaattaaacgaccacatatggttagggctagtggctcccacattggatagggcagatgtggagctgatgtagcaccacagtgtaaagtgtttgtcatccaaaaaatccagatgcccagtccctccatctcagagactgcagaatgatggagaccacttgaggtcatcttatccaatcccctccttgcagtggagaaactgaggcacaaagagaggagctgacttccccgaggtcacagagcaagtgggcaagctggagcccactgggccaggtttcctggctcccagacaagtgctctttccaggacctgtccgcctcctgccttttataatcccacaccagactctgggtacaactcagttcaggttgagtatgcttttttaactttcacatatctgaacagtccactgtggcagaacaccttaaatatccaagggaggttgcctgtgtcagccaaaaaggaaatacaagcccacaattcaccacttctctcctgggtggcttgcgcagcatggtggtgacaagggcccaggccagcttgagctccaccaccccaggtgacaaaaggggaagccagagcttacccaagcagagccctgccctggtgctgcccttcccagggtccagccaagaatgtggagaggctgcagcatgatggacaaggcgggggacatatgtcacagctacagaggtcggggtgggctccaagccctgggtcactcacttgccccaggtagggaagactgaaacacaaatgccctgcccaagaacaggacagagttgagacttaccaaagctcacgctgagttcactgctttacagaggccccttttcttggctggactgccagatggttcttagtagacccagggaactctatgctttcttaaaaagcctggaattcagttttggtcaaggccgttgatgtagcgcatggtgacttcacagtggccccacacggcactcaccaccgggtacagcttcttgcccttgagacctcggaaggccacgcccaggtactggccatccacgatgaagctgagtgtgccctcatccatgtccagcaccacgagcagcgagtcgggcagcgcaaaggcctcgtcgggccccagaaaggccgggtaggccacgccgggctggttcttgccgtcgtggtagaggcggctgcggcccaggtcccagccccacgactcggcgtcactgcctaccagcgccgtgtagcccacggagtgcaggggagcacgggccgtggccacaccaactacagcgtgggtgccgcgctgccgagccggccagttgatctgccaggcgtgcaggccgcgggcgtggcccaccttgccgcggatgccgtcggtgctctgggccacggggtgccggtggaaggtgagccggtcgtcgtccttgacgaagacgttgagcgagcggtcctcggggttccacgcgtgccgcagctgcacagccagccccgccgctggcatgtccaacagctggtccagccgcgccggccgcccgggctctgcaccccgcagctcccgcttggccggccgcagcgccggctctcgcacctccactgacttgaggctccccgagagcttctggcccatgcttcactgcggggaggaggccgctgcaggccaccgctacctcgtgggagcctccactccccgtagccaggaatgggccacggggctgggaaccaggcttccggacggtagacctccacagcctctaccgggctgcggcaggggcccaagctccataaaagagagggcaagcgcctgttcgggaagaatccccagcgctggcaggtcctggactc

SEQ ID NO: 16284 - RNA, 1690 nt, Homo sapiens
  source 1..1690: mol_type = other RNA
ggctcatgtgtctgtcctcttctcctgaatatgggtggttggtgcgggggcagggggtgagtcactgcactgtttcccatgcctcccacctcggctctcatggttgggagcggctgagggaggaggctgaggcagggagagggaagacccaggagggaggaggcaggcgctgctttgaggggtgccctggagccttggcaatccttttcctcctcgggcccgggagcccaggccccgtctccaccagccgcaggcgacagctgtcatggtggtctacagcctgggcctggggaagggctcagagcagtgtgcagctgcagccttgggcctccatggccaccagcagcatcctcaggcggcgcggcgattgcggcgggtagcggagggcgttgagcttctccatccccgggctgcgcaggaggcaggcgcgatggtgggagaaggtgtcgaaggagaacttgccatggtaccggcccatcccactggcacccactcctccaaaaggcaggctggccagggtcatgtgcatgaagccgtcgttcccacagaagcccccgctgctggtctgggtcagcacccgcttgaccacctggctgctgttggagaaggcgtacagggccaggggcttctcccgccggttgatgaactcgatggcctcgtccaagctctgcacgttcacgatgggcaggatgggcccgaagatctcctcctgcatcacaggctccatctcctgcacatccaccagcaccgtgggggcgatgtagcgatcgctctcatcgctctggcccccaatggccacacggccgcagcccagcaatgcccgcagccgctggaactgtttctggttgatgatgcggcccaggtttggggagctctgggggtcgtcgccatagaaacgggtgatggtgctctgcagggcaggcagcagcctctcctgcatctcagggctgcataggacgtagtcgggggccacgcaggtctggccggcgttgaagtagcggaaccaggccacgcggttggccacggtctgggggtcgcagttgtcgtccacgtagcaagggttcttgccccccagctccagggtgacaggtgtcaggtgcttggcggcagcagtcataacaatcttgcccacacgagggctccctggtccacgtattggggcagcacctcggccaggatcttctcgacgttcttgctaatctccgatggcttcagcaccacacagttccctgcagcgagggctcccacgaggggcaccagcgtcaggttcagcggatagttccagggcgcaatgatgaggaccaggccaaagggctccttccggatgaaggcggagtccagctgcgtggccaggttcttgggcacacgctcgtccttcatccaggcccggaggttcctgagggccagggtgacctcgccctggctgatggcaacctcagacacctccgactcgaaggctgacttgtgcaggtcctgggccagtgcgtcgtgcagaagctgcttgttttcttgcaggaagcggcccaggccttggagctgcgcagcccggaactcagctggccgcgtgcgccccgcgtggaaggcctcccgcagtcgccgcagcgtgtccccaagggggtccatcctgaggctctgccaagctgcccttcctcctggctgtcccgctctgcctggtggccctgctgttaag

SEQ ID NO: 16285 - RNA, 1772 nt, Homo sapiens
  source 1..1772: mol_type = other RNA
ggctcatgtgtctgtcctcttctcctgaatatgggtggttggtgcgggggcagggggtgagtcactgcactgtttcccatgcctcccacctcggctctcatggttgggagcggctgagggaggaggctgaggcagggagagggaagacccaggagggaggaggcaggcgctgctttgaggggtgccctggagccttggcaatccttttcctcctcgggcccgggagcccaggccccgtctccaccagccgcaggcgacagctgtcatggtggtctacagcctgggcctggggaagggctcagagcagtgtgcagctgcagccttgggcctccatggccaccagcagcatcctcaggcggcgcggcgattgcggcgggtagcggagggcgttgagcttctccatccccgggctgcgcaggaggcaggcgcgatggtgggagaaggtgtcgaaggagaacttgccatggtaccggcccatcccactggcacccactcctccaaaaggcaggctggccagggtcatgtgcatgaagccgtcgttcccacagaagcccccgctgctggtctgggtcagcacccgcttgaccacctggctgctgttggagaaggcgtacagggccaggggcttctcccgccggttgatgaactcgatggcctcgtccaagctctgcacgttcacgatgggcaggatgggcccgaagatctcctcctgcatcacaggctccatctcctgcacatccaccagcaccgtgggggcgatgtagcgatcgctctcatcgctctggcccccaatggccacacggccgcagcccagcaatgcccgcagccgctggaactgtttctggttgatgatgcggcccaggtttggggagctctgggggtcgtcgccatagaaacgggtgatggtgctctgcagggcaggcagcagcctctcctgcatctcagggctgcataggacgtagtcgggggccacgcaggtctggccggcgttgaagtagcggaaccaggccacgcggttggccacggtctgggggtcgcagttgtcgtccacgtagcaagggttcttgccccccagctccagggtgacaggtgtcaggtgcttggcggcagcagtcataacaatcttgcccacacgagggctccctgtgaagaagatgtagtcgaacctgtgctctagcagctgccccgtctcctggggcccgcccagcaccacagcaaagcagctctggtccacgtattggggcagcacctcggccaggatcttctcgacgttcttgctaatctccgatggcttcagcaccacacagttccctgcagcgagggctcccacgaggggcaccagcgtcaggttcagcggatagttccagggcgcaatgatgaggaccaggccaaagggctccttccggatgaaggcggagtccagctgcgtggccaggttcttgggcacacgctcgtccttcatccaggcccggaggttcctgagggccagggtgacctcgccctggctgatggcaacctcagacacctccgactcgaaggctgacttgtgcaggtcctgggccagtgcgtcgtgcagaagctgcttgttttcttgcaggaagcggcccaggccttggagctgcgcagcccggaactcagctggccgcgtgcgccccgcgtggaaggcctcccgcagtcgccgcagcgtgtccccaagggggtccatcctgaggctctgccaagctgcccttcctcctggctgtcccgctctgcctggtggccctgctgttaag

SEQ ID NO: 16286 - RNA, 1852 nt, Homo sapiens
  source 1..1852: mol_type = other RNA
ggctcatgtgtctgtcctcttctcctgaatatgggtggttggtgcgggggcagggggtgagtcactgcactgtttcccatgcctcccacctcggctctcatggttgggagcggctgagggaggaggctgaggcagggagagggaagacccaggagggaggaggcaggcgctgctttgaggggtgccctggagccttggcaatccttttcctcctcgggcccgggagcccaggccccgtctccaccagccgcaggcgacagctgtcatggtggtctacagcctgggcctggggaagggctcagagcagtgtgcagctgcagccttgggcctccatggccaccagcagcatcctcaggcggcgcggcgattgcggcgggtagcggagggcgttgagcttctccatccccgggctgcgcaggaggcaggcgcgatggtgggagaaggtgtcgaaggagaacttgccatggtaccggcccatcccactggcacccactcctccaaaaggcaggctggccagggtcatgtgcatgaagccgtcgttcccacagaagcccccgctgctggtctgggtcagcacccgcttgaccacctggctgctgttggagaaggcgtacagggccaggggcttctcccgccggttgatgaactcgatggcctcgtccaagctctgcacgttcacgatgggcaggatgggcccgaagatctcctcctgcatcacaggctccatctcctgcacatccaccagcaccgtgggggcgatgtagcgatcgctctcatcgctctggcccccaatggccacacggccgcagcccagcaatgcccgcagccgctggaactgtttctggttgatgatgcggcccaggtttggggagctctgggggtcgtcgccatagaaacgggtgatggtgctctgcagggcaggcagcagcctctcctgcatctcagggctgcataggacgtagtcgggggccacgcaggtctggccggcgttgaagtagcggaaccaggccacgcggttggccacggtctgggggtcgcagttgtcgtccacgtagcaagggttcttgccccccagctccagggtgacaggtgtcaggtgcttggcggcagcagtcataacaatcttgcccacacgagggctccctgtgaagaagatgtagtcgaacctgtgctctagcagctgccccgtctcctggggcccgcccagcaccacagcaaagcagctctggtccacgtattggggcagcacctcggccaggatcttctcgacgttcttgctaatctccgatggcttcagcaccacacagttccctgcagcgagggctcccacgaggggcaccagcgtcaggttcagcggatagttccagggcgcaatgatgaggaccaggccaaagggctccttccggatgaaggcggagtccagctgcgtggccaggttcttgggcacacgctcgtccttcatccaggcccggaggttcctgagggccagggtgacctcgccctggctgatggcaacctcagacacctccgactcgaaggctgacttgtgcaggtcctgggccagtgcgtcgtgcagaagctgcttgttttcttgcaggaagcggcccaggccttggagctgcgcagcccggaactcagctggccgcgtgcgccccgcgtggaaggcctcccgcagtcgccgcagcgtgtccccaagggggtccatcctgggagggcggtgaggtcttctggaccatgcccacaccggtggcccgtgattagatagttagggtgggggtgaaggactgcagagcccctgtcctctgtgtgggatggagcccccagccactgccagtcacgtggctcagcatgt

SEQ ID NO: 16287 - RNA, 1661 nt, Homo sapiens
  source 1..1661: mol_type = other RNA
ggctcatgtgtctgtcctcttctcctgaatatgggtggttggtgcgggggcagggggtgagtcactgcactgtttcccatgcctcccacctcggctctcatggttgggagcggctgagggaggaggctgaggcagggagagggaagacccaggagggaggaggcaggcgctgctttgaggggtgccctggagccttggcaatccttttcctcctcgggcccgggagcccaggccccgtctccaccagccgcaggcgacagctgtcatggtggtctacagcctgggcctggggaagggctcagagcagtgtgcagctgcagccttgggcctccatggccaccagcagcatcctcaggcggcgcggcgattgcggcgggtagcggagggcgttgagcttctccatccccgggctgcgcaggaggcaggcgcgatggtgggagaaggtgtcgaaggagaacttgccatggtaccggcccatcccactggcacccactcctccaaaaggcaggctggccagggtcatgtgcatgaagccgtcgttcccacagaagcccccgctgctggtctgggtcagcacccgcttgaccacctggctgctgttggagaaggcgtacagggccaggggcttctcccgccggttgatgaactcgatggcctcgtccaagctctgcacgttcacgatgggcaggatgggcccgaagatctcctcctgcatcacaggctccatctcctgcacatccaccagcaccgtgggggcgatgtagcgatcgctctcatcgctctggcccccaatggccacacggccgcagcccagcaatgcccgcagccgctggaactgtttctggttgatgatgcggcccaggtttggggagctctgggggtcgtcgccatagaaacgggtgatggtgctctgcagggcaggcagcagcctctcctgcatctcagggctgcataggacgtagtcgggggccacgcaggtctggccggcgttgaagtagcggaaccaggccacgcggttggccacggtctgggggtcgcagttgtcgtccacgtagcaagggttcttgccccccagctccagggtgacaggtgtcaggtgcttggcggcagcagtcataacaatcttgcccacacgagggctccctgtgaagaagatgtagtcgaacctgtgctctagcagctgccccgtctcctggggcccgcccagcaccacagcaaagcagctctggtccacgtattggggcagcacctcggccaggatcttctcgacgttcttgctaatctccgatggcttcagcaccacacagttccctgcagcgagggctcccacgaggggcaccagcgtcaggttcagcggatagttccagggcgcaatgatgaggaccaggccaaagggctccttccggatgaaggcggagtccagctgcgtggccttgtgcaggtcctgggccagtgcgtcgtgcagaagctgcttgttttcttgcaggaagcggcccaggccttggagctgcgcagcccggaactcagctggccgcgtgcgccccgcgtggaaggcctcccgcagtcgccgcagcgtgtccccaagggggtccatcctgaggctctgccaagctgcccttcctcctggctgtcccgctctgcctggtggccctgctgttaag

SEQ ID NO: 16288 - RNA, 1421 nt, Homo sapiens
  source 1..1421: mol_type = other RNA
ggctcatgtgtctgtcctcttctcctgaatatgggtggttggtgcgggggcagggggtgagtcactgcactgtttcccatgcctcccacctcggctctcatggttgggagcggctgagggaggaggctgaggcagggagagggaagacccaggagggaggaggcaggcgctgctttgaggggtgccctggagccttggcaatccttttcctcctcgggcccgggagcccaggccccgtctccaccagccgcaggcgacagctgtcatggtggtctacagcctgggcctggggaagggctcagagcagtgtgcagctgcagccttgggcctccatggccaccagcagcatcctcaggcggcgcggcgattgcggcgggtagcggagggcgttgagcttctccatccccgggctgcgcaggaggcaggcgcgatggtgggagaaggtgtcgaaggagaacttgccatggtaccggcccatcccactggcacccactcctccaaaaggcaggctggccagggtcatgtgcatgaagccgtcgttcccacagaagcccccgctgctggtctgggtcagcacccgcttgaccacctggctgctgttggagaaggcgtacagggccaggggcttctcccgccggttgatgaactcgatggcctcgtccaagctctgcacgttcacgatgggcaggatgggcccgaagatctcctcctgcatcacaggctccatctcctgcacatccaccagcaccgtgggggcgatgtagcgatcgctctcatcgctctggcccccaatggccacacggccgcagcccagcaatgcccgcagccgctggaactgtttctggttgatgatgcggcccaggtttggggagctctggtccacgtattggggcagcacctcggccaggatcttctcgacgttcttgctaatctccgatggcttcagcaccacacagttccctgcagcgagggctcccacgaggggcaccagcgtcaggttcagcggatagttccagggcgcaatgatgaggaccaggccaaagggctccttccggatgaaggcggagtccagctgcgtggccaggttcttgggcacacgctcgtccttcatccaggcccggaggttcctgagggccagggtgacctcgccctggctgatggcaacctcagacacctccgactcgaaggctgacttgtgcaggtcctgggccagtgcgtcgtgcagaagctgcttgttttcttgcaggaagcggcccaggccttggagctgcgcagcccggaactcagctggccgcgtgcgccccgcgtggaaggcctcccgcagtcgccgcagcgtgtccccaagggggtccatcctgaggctctgccaagctgcccttcctcctggctgtcccgctctgcctggtggccctgctgttaag

SEQ ID NO: 16289 - RNA, 36 nt, Homo sapiens
  source 1..36: mol_type = other RNA
ggctcctcctctcaggatgtggagctggaagactgt

SEQ ID NO: 16290 - RNA, 651 nt, Homo sapiens
  source 1..651: mol_type = other RNA
ggctgagtggggttctgactccccagtcaaggatgagttgtccaccttacatccttgtgcagagataagccggaggtcagcagggactcggtctccacccttgatttccaccaggtctcccaacaccacctcttgtacattaatttgcatcttctctcctcctcgaattaccagagcttgctgaggcaccatgttcttaaaagactccatgatcttggagctcttggcctcctgataataggagaagcagccagtgacgatgaccacgacggacagtacgatgctcaggtagaggttgtctttggtaggctcctcattgaaatatatctggatgctgtaggccacaaagcagagaatggccccagtccatagtaggagggagaagcctccgaacagttgcttacagaatttgacccattctggagtggtggggggtggggtaacagtattgggtccacctcgagtcaggatttcctttgccctttggtggctatggcccatttgcagctttttccaggtagtgtccatggaacgtggccaggcagagggtgaggggtgggaacgttggacttgaagttagggggctggattcctagttcagcttttgtcctggcagcctcacagtcagagttggagactctctgcctcctc

SEQ ID NO: 16291 - RNA, 1143 nt, Homo sapiens
  source 1..1143: mol_type = other RNA
ggctgagtggggttctgactccccagtcaaggatgagttgtccaccttacatccttgtgcagagataagccggaggtcagcagggactcggtctccacccttgatttccaccaggtctcccaacaccacctcttgtacattaatttgcatcttctctcctcctcgaattaccagagcttgctgaggcaccatgttcttaaaagactccatgatcttggagctcttggcctcctgataataggagaagcagccagtgacgatgaccacgacggacagtacgatgctcaggtagaggttgtctttggtaggctcctcattgaaatatatctggatgctgtaggccacaaagcagagaatggccccagtccatagtaggagggagaagcctccgaacagttgcttacagaatttgacccattctggagtggtggggggtggggtaacagtattgggtccacctcgagtcaggatttcctttgccctttggtggctatggccctttgtcaggtccacggagtacttggtgctcagctcttccaaggttaatttgtgatcatccatgaccacttccttcttcagttcctccatattgcgcttctgtttttccctcttcaccatttttttcttgataagcccttttttaggtcttcgtcttggactctggtcatggggagccactgtccctttcttcccccaaagccccatagctatccccagaaagagctgcccgagctcaactgtgggaagaaagctgagagagtgaggcaaggggaagggaagagggcgcgcgggcaagggggccacgagaagagagtggtggggagagaatgagggagcagaaagaaagaggcagggagggaggtgttgggtggtgaaggtgagagagaggaagggaagtgagagaggagagactgagcggtcctccagccgtccgctgggaagaggaagagtcaggagtgagggaagagggaggagagaagcctagggtggaaggataaaaaggtagaggtgagggaatgcagtgagggcaggaaacaagaggtgaagcgtaaccaggtgcctcagtgatgaagatgccgcaaggcccacaggaaggtgggaaatgcagtgagagtgaggaggcggagtgagcttcaaggatct

SEQ ID NO: 16292 - RNA, 1833 nt, Homo sapiens
  source 1..1833: mol_type = other RNA
ggctgggtgctcttgtgcagtcacatcgtcttacaggaaggggaaaaaacagttctgttcaaaacaactcaccaggttctgacaataacaaagaacaacatggggctgagatttgagtagggaataaactgagtgcagacaaatcatataattaaattaaacggtatccctgaaaataaaaagaacaatttcaaaactcacaagtagaagggaggccttggtaattatttttaaaaatgttcattaagctccaatgattgtttgctgctatccttatctacagtcatgctgagtaaagctatagctaaatggaagttaaattgtattcacgaggtgttaatgtttacatcttattatctgcagtctctcagagaaagcaaaagtaactacaaatagcgctatgccagaaactggtttcttgaccaacaatgtcgcttcagcatgcaatgaactggttcattctaaagtggtcacggctgttgatgacaagaggctttgtatttttatatggcacatcttttggtccatgtgaaaacaagttttttgaatgttaactattttctgacactttggagttactgttgctcttcccatttccattaggtcgatatatggttcatggcaatactgtacaagtttaaaatttcattacaggaagtagtctggggtacgacgagtaacatgtggctcgcctctacgaggtgctgggtcaaactgcaagaaagagtattttagagtatcgtcaagttccatgattgcagcttggttaccacaacgataacaatagtttggagcactgaaaatcgttactacattccggtcatggcaccagttatatccctccatcactagctggtgagctctagacaccaacgtgaggccattggcatgattaaatgtctcagaaatatcttgcccaaaggtgtaaccagctcctcgaggagatataccccaaccaccacggtcatctggatctgaccacagcaagtcacacattggaccctaaaaaataactcatggggaacttcttgtaggcgatcaagtgctctgatatgatccagtgtatctatagatggcgagagaccaccatgtagacagaagatctgcccatccaccaaggcagtgagaggaagatagtcaaaaagatctgtaaaatatttccaaacatttgcatttccatattttcttaaacattcatcatagaaaccataaacttgtgtgatctgtctgctctcatgattccctcgaagaatggtgatgcgttcacggtaacgaaccttaagagctacaagcagtgtaactgtttcaactgaataatatcctctgtcaacataatctcccataaacaagtaatttgtatctggtgatttgccaccaattctaaacagttccatgagatcatgaaattgcccatgcacatctccacagacagtaactggacatcgaacctcttgcacgttggattcttttgtcaggatttctttagccttgatttctggagaagatcgcttggtgagtttaatacaaaccaccaaggggtactaaagctgtgtgacctttaggtatgttctgggatacggcctaacaagactgcctttgggggatcctctgggcagctctggacctaactaggcctgggtaccagcggcaagactcttactcagcccaccggagaggcccaggctccattcccaagccgcagaatccaagccagctcaccctcaaaaccgtccctgacgatgacccacagggtctccgctccccctgccacctcgtctggcgccaaggccggctgactcaaaagcccaggagtcgagtgaacggcgccatttt

SEQ ID NO: 16293 - RNA, 1790 nt, Homo sapiens
  source 1..1790: mol_type = other RNA
ggctgggtgctcttgtgcagtcacatcgtcttacaggaaggggaaaaaacagttctgttcaaaacaactcaccaggttctgacaataacaaagaacaacatggggctgagatttgagtagggaataaactgagtgcagacaaatcatataattaaattaaacggtatccctgaaaataaaaagaacaatttcaaaactcacaagtagaagggaggccttggtaattatttttaaaaatgttcattaagctccaatgattgtttgctgctatccttatctacagtcatgctgagtaaagctatagctaaatggaagttaaattgtattcacgaggtgttaatgtttacatcttattatctgcagtctctcagagaaagcaaaagtaactacaaatagcgctatgccagaaactggtttcttgaccaacaatgtcgcttcagcatgcaatgaactggttcattctaaagtggtcacggctgttgatgacaagaggctttgtatttttatatggcacatcttttggtccatgtgaaaacaagttttttgaatgttaactattttctgacactttggagttactgttgctcttcccatttccattaggtcgatatatggttcatggcaatactgtacaagtttaaaatttcattacaggaagtagtctggggtacgacgagtaacatgtggctcgcctctacgaggtgctgggtcaaactgcaagaaagagtattttagagtatcgtcaagttccatgattgcagcttggttaccacaacgataacaatagtttggagcactgaaaatcgttactacattccggtcatggcaccagttatatccctccatcactagctggtgagctctagacaccaacgtgaggccattggcatgattaaatgtctcagaaatatcttgcccaaaggtgtaaccagctcctcgaggagatataccccaaccaccacggtcatctggatctgaccacagcaagtcacacattggaccctcatggggaacttcttgtaggcgatcaagtgctctgatatgatccagtgtatctatagatggcgagagaccaccatgtagacagaagatctgcccatccaccaaggcagtgagaggaagatagtcaaaaagatctgtaaaatatttccaaacatttgcatttccatattttcttaaacattcatcatagaaaccataaacttgtgtgatctgtctgctctcatgattccctcgaagaatggtgatgcgttcacggtaacgaaccttaagagctacaagcagtgtaactgtttcaactgaataatatcctctgtcaacataatctcccataaacaagtaatttgtatctggtgatttgccaccaattctaaacagttccatgagatcatgaaattgcccatgcacatctccacagacagtaactggacatcgaacctcttgcacgttggattcttttgtcaggatttctttagccttctcgcagaggctcttgacctgggactcggacagctgcttgcactcgttcagctgctcgatccactggtccagctccttggtgaacaccttctcgtccatgatgccacccgccccagccggctgccgctccgcgctgctcccgcgccgccgcccgcacacgggcctacacgcacacgccgccgccggttcctcgtgtacttctggcggctgttgaggctggcgctggcccgctggctctcaccgcagtactcggccgtcggccgctgcgcctcctcctccgctcgctgaggctccagagctcggctctctgt

SEQ ID NO: 16294 - RNA, 1822 nt, Homo sapiens
  source 1..1822: mol_type = other RNA
ggctgggtgctcttgtgcagtcacatcgtcttacaggaaggggaaaaaacagttctgttcaaaacaactcaccaggttctgacaataacaaagaacaacatggggctgagatttgagtagggaataaactgagtgcagacaaatcatataattaaattaaacggtatccctgaaaataaaaagaacaatttcaaaactcacaagtagaagggaggccttggtaattatttttaaaaatgttcattaagctccaatgattgtttgctgctatccttatctacagtcatgctgagtaaagctatagctaaatggaagttaaattgtattcacgaggtgttaatgtttacatcttattatctgcagtctctcagagaaagcaaaagtaactacaaatagcgctatgccagaaactggtttcttgaccaacaatgtcgcttcagcatgcaatgaactggttcattctaaagtggtcacggctgttgatgacaagaggctttgtatttttatatggcacatcttttggtccatgtgaaaacaagttttttgaatgttaactattttctgacactttggagttactgttgctcttcccatttccattaggtcgatatatggttcatggcaatactgtacaagtttaaaatttcattacaggaagtagtctggggtacgacgagtaacatgtggctcgcctctacgaggtgctgggtcaaactgcaagaaagagtattttagagtatcgtcaagttccatgattgcagcttggttaccacaacgataacaatagtttggagcactgaaaatcgttactacattccggtcatggcaccagttatatccctccatcactagctggtgagctctagacaccaacgtgaggccattggcatgattaaatgtctcagaaatatcttgcccaaaggtgtaaccagctcctcgaggagatataccccaaccaccacggtcatctggatctgaccacagcaagtcacacattggaccctcatggggaacttcttgtaggcgatcaagtgctctgatatgatccagtgtatctatagatggcgagagaccaccatgtagacagaagatctgcccatccaccaaggcagtgagaggaagatagtcaaaaagatctgtaaaatatttccaaacatttgcatttccatattttcttaaacattcatcatagaaaccataaacttgtgtgatctgtctgctctcatgattccctcgaagaatggtgatgcgttcacggtaacgaaccttaagagctacaagcagtgtaactgtttcaactgaataatatcctctgtcaacataatctcccataaacaagtaatttgtatctggtgatttgccaccaattctaaacagttccatgagatcatgaaattgcccatgcacatctccacagacagtaactggacatcgaacctcttgcacgttggattcttttgtcaggatttctttagccttgatttctggagaagatcgcttggtgagtttaatacaaaccaccaaggggtactaaagctgtgtgacctttaggtatgttctgggatacggcctaacaagactgcctttgggggatcctctgggcagctctggacctaactaggcctgggtaccagcggcaagactcttactcagcccaccggagaggcccaggctccattcccaagccgcagaatccaagccagctcaccctcaaaaccgtccctgacgatgacccacagggtctccgctccccctgccacctcgtctggcgccaaggccggctgactcaaaagcccaggagtcgagtgaacggcgccatttt

SEQ ID NO: 16295 - RNA, 43 nt, Homo sapiens
  source 1..43: mol_type = other RNA
ggctggtcagatgggagtgagccctgggcagcccccaggcccc

SEQ ID NO: 16296 - RNA, 1406 nt, Homo sapiens
  source 1..1406: mol_type = other RNA
ggctggtcagatgggagtgcaggtgcagaagacgccgtgagcaaagatgcacaagagatgatggccccaaactggaaccagcccaggaggatgcagggaagggcggatgggagctgggaagacagaccccagcgaccaggtggagccacaccagcagggcacctggagtcaagctaacctggtgcaccagaggatggaggacgcagcgcccatcgtggggtgcagagggaacctcgggcaaggcagcggtgcccctccccactggacagccaagctgggctgggagcaggcccttcagccagcagagttgcagagtgaaccctgggctccggggaggaagaggtgaatcagacccagccctgcccttggggactcgcctcctcgtagggtagatggagctttaacagatggtccccatggggctgggccagatgctgaggacacagcggcagatgatcacctggcactgggggcgtcatctgaagcgagctcagatgaagaggtgaactcacaggccgtgaggagtgacccacttgaggagggctggagtggggcttgaactgggcgtgtctgcttccaagcctgtggtgcgcttgaccatccccccttcctgctgtgttcactgactccagatgttcccaggccttgccctcgaggagctccccatgtggccaggagaccatcacaagccagtgcccagcgctgagggtagggggagtgggccccctcccaggtcacagaggactcctgggtgtgagaaaggtgacatcagaactgggcgtggagaacaagacatggctttccaggcagagaacaggaaacgcaagggtctgccgggaacagcacgcagttgtcgaggagaagagaggggccactgcatgcctggcgggtgctgggcgggccgtggggtgaggctggggcatgtggtagagaccaggaagcagccaggtgggcccagccagacctgaggacccctcatccctgccaaggaggcttgtgcttgatcctgtcgacatcagaagaaagagggattgggtggcgggtacccgtcaaaagaaagagggattgggtggcgggtacccgtcagacctgaaatgcgtgagtgtccgggagggaggaggccagtgggaagctaagccttgagctgcctgaggccatatgcagggaggacagagcctgggacagccaccgaggtctcagtgcctcctagggttcctctaccccatgcatcaaagcacaacctcgctctcccacaccatctgcctgagcagggtttcctgtgcgctggggctggaccccatatctaatgttcctggatggagtcccaggaaaacaattttgcttatttatcacacacacacacacacacacacacacacacacacgcacacacagcaacatcataa

SEQ ID NO: 16297 - RNA, 51 nt, Homo sapiens
  source 1..51: mol_type = other RNA
ggcttctttacagtgctgccttgcgttctgtggagaagactagagaggacc

SEQ ID NO: 16298 - RNA, 60 nt, Homo sapiens
  source 1..60: mol_type = other RNA
ggcttctttacagtgctgccttgtagcattcaggtcaagcagcattgtacagggctatga

SEQ ID NO: 16299 - RNA, 60 nt, Homo sapiens
  source 1..60: mol_type = other RNA
ggcttctttacagtgctgccttgttgcatatggatcaagcagcattgtacagggctatga

SEQ ID NO: 16300 - RNA, 305 nt, Homo sapiens
  source 1..305: mol_type = other RNA
ggcttgcatgggggactgggcccgcacacgcccccggagcggtagccgaagctgcgtccgcaggagccggcccgaaagcctccgcacacgctgtggctgccgaagcccccggtgaggccgcggtagcaggagatgccacggtagggggcggcggtgatgcagcagcggccgggccgcggcccgcaggccgagatgcagctgaaggcgcgcccaccaaatcctgatccgcaggtcatgatcctcctggacgtttgggttgcagaggacaggataggggacctggagtcctgatggaaactccaatg

SEQ ID NO: 16301 - RNA, 444 nt, Homo sapiens
  source 1..444: mol_type = other RNA
ggcttgcatgggggactgggcccgcacacgcccccggagcggtagccgaagctgcgtccgcaggagccggcccgaaagcctccgcacacgctgtggctgccgaagcccccggtgaggccgcggtagcaggagatgccacggtagggggcggcggtgatgcagcagcggccgggccggggcccgcaggccgagatgcagctgaaggcgcggccaccacagtaagatccacaagtcatggtgctgactctcagcactgcccacctccaccgtcagccactggatggcctgattaagcctgttcagatcctccttgctgggcttcaggctctgcgtgtgtttctgcacagttgcctttaattcctcacacatggagaaagaactgtggtctcctccaagcctctcttgagcaccaaagcccagcttcagcccaagagctaccagaat

SEQ ID NO: 16302 - RNA, 4680 nt, Homo sapiens
  source 1..4680: mol_type = other RNA
ggcttgcatgggggactgggcccgcacacgcccccggagcggtagccgaagctgcgtccgcaggagccggcccgaaagcctccgcacacgctgtggctgccgaagcccccggtgaggccgcggtagcaggagatgccacggtagggggcggcggtgatgcagcagcggccgggccggggcccgcaggccgagatgcagctgaaggcgcggccaccacagtaagatccacaagtcatggtgctttttggggaagagaggaggttctgaggatggagacgtccgaatggagagcacagtggtcggggcgtcaggcgttcactacttgcacctctgtaggcctgactctcagcactgcccacctccaccgtcagccactggatggcctgattaagcctgttcagatcctccttgctgggcttcaggctctgcgtgtgtttctgcacagttgcctttaattcctcacacatggagaaagaactgtggtctcctccaagcctctcttgagcaccaaagcccagcttcagcccaagagctaccagaatccttgccactgaggactagggcctcttcttcctgggggctctgtgacctcatctcattacaatcacagagttctgcccaggaggcctcaggggcatagggtagaagagggccatactctgaccccaggtgggaaaatggaagtttctgggctgaagtggaacttaaaggaaagtggaggaggggaaggctacctcaggtggaggaaatgtgtggagctgaggagcttaggcttatggatgggcactggggagccacagagggtgtctgagcaggacagtggcctgacatgagatgtgattgtctagaagcagtgcagaagattgacaggagggcaagaaattgggactggggatgccagtcccaagacttggtaggaaatcttgggtagggcaatgactttaacctgtaggaatgagtaggggctagagagcacaagctgtggtcagcattttctttttgttttataaatttctcatatatgcaaaagagtatgcaaaacctacatttattgatttcaatagcaacaataataaaacaaatccttgtgtacccaccagtaccttcaaagccccctgcgggatttttgctgatccatctccaaccccatctgatccccaaagtaaccactgtcctgagtttttatattggtcattcccttgcttttctttattactatgtcataacgtgtatccataaactagtgttgagttttgcctacctttaagttttatataaatagaattacaccttgtacatttctatgacttgctttttcctcctcaacatactagttttgagattcatctttttgatgcatgtagttttatttctcagtgttgtatagtattccaaagtatgactacatatatatagatagatacagatatagacacacacatatacatatatctctattttcctataggtagcacatgtgttttttgtttttgttgtaacaaacaatgctgccatgaactttcttgtacatatctgctggtggacctcaacaagaggttctttggggtactagttgtcaaactgttttttaacctcaactctaaataagaaatatatgttgtatcatgaatcactacctacgtacaaatacaccacatctactgaaataagtttcatggaaaaatcatttacttctactatgtgtaaggcaatctgatctaaccaatcaccttaacacattcttttactttcaacttatgtcctcatgttttaagtttatttcttataactagcatattactttattattataatataatgaaaatgaaatactcatgaacctacttactgatcccaaaactaaaatcttactagtaatttacatttagctccatgctccttccctaccctgtcctctcctaaccaccccagaggtaaccacttccctaaagttgatataattcctttgttttttcttagctttatcaaatacatgcatatgcctcaatatatatttgtttcagtttttttgttctttttttataaaaagtgtgtcacacagggtcttgttttattcaacattatgttgctagtattcctccattataatattaatattccattcttatagtattccattgtgtaactataccacactttaggtaattctattactgttttgttttgtttctttctcttacaaaggtggtgccatgaacatttttctacatgtcctccgatgcacatatgtgaggatttgtatacaactacaaacagaacttctgactcataggatggtcagaatcttataaaggtgttaactttataagataatataaaattattttccaaagttgttataacaattcacactttgctcagcaatgtgaaaaagattcgtatcctctttaatgtgtcttaattttcaacaattaaataatgcaatctcatttttggtcttgctttgtattttcatgattactgttaaagtttaatatctctttaaatgtctattacatgtgtatttccttttcttttgtccatttttttctattgggtttttgctgtattctaaaggattataagtgttctttatatttctgagtattactattatatcacttacatatatcacaaatattatcaagtttacagcttatcttttcactttatcacctattttgaaaaataaagttgttagttttaatgtaatctaatttatcaatcttttatgttgagcattttatgtgacatgtttaaaaatccttctctacaccaaggtcagaaaaatattctccaatattttcttctaaaattcttaaagttttgcttttgacatttgtaatttaaattaatttgaaactgattttgtgtataagagaaaacagggatctaattttattttttacatgtggttaaccaatgcatagtccttttcactactgatctgccataccacttctattttacaacaaaatcatttacttatttataaataaatttaggggctattttgttccattggtcagtttgtctatttttgtgtgggtactatactttctcaattactataactctataatacattataatccctgaaagagagagtacctatttcttccttctcatcattccttagctgttcttgacctttgttcttccccataaattttagaatcaacttgtcaagaattatgtaaatcttcatttggaatttgagtgtagttgcgtcaactctgtagatcactgtaaggataattaacatattcatgatagtaaagcttcctatctaagaacatggtatagctcttcatttaattatgtcttctttatcttttctttcctataacattttgtgtaacgcttatatttctctaggtgtaagtctttcacatatgtgttagatttatttctaagtatcttatgcattttaaatcattattttatcaacttaattgacatataatttgcatacaattgtatctcaataaagcgcacacattctaaaagtacagttcaacaaattttgacagatgtatgctccaatctaatcaccactgaatgaatctagttcattattttttgttgctgaatgatattttattgtatgactatatctcaatttgtttatccattcatctgctggtacacatttgggttgtttccaatttagggctattataaataaagcttctataaaattcatgtacaagtctctgtatagatctgcttttatttcttttgagcaaatacccaggagtggaattgctgcatcatttgataagtgcatgtttaacttcataagaaattgccaaactgttttccaaagttgctcaatcattttacactccacaaaagtttcagctgattcacacttggtattgtcagtctattaaattttagccttctaaaggaggcaagaagcaaggaggaaaagaagaccagagaagggaagggaagagcaagacagcaagggaagcagaaggttgaaagatggttggtgagaggctatcctcttcgtgggttcagtcaggtcagaatcctcaaacagaacatgcccatgggctacgtgccactcctctcaatagcctttctcagcttgagggcagcaggggccaaggaagagagattcccacacaacaagaagtaagaagtgggaagcagacaacgtggatcagggtgggtcaagcagtggcgccctgccaccaggctgcacaaggtcaggtagggccagctgggaccctcgcaagggtgagaggctgggctgggtgcatcctcaagctctgccaacttaacacttcctgtagctgctgccacaggccccatcccacaggagctgatgccgcaggtgcaggtggccaagaggcccccacaggcaaccccaccaaggagctgctcacacctgcacagagacagccataagaagttaaaccctttggtcggggtgggagctggtcccaaaaagccccacctccaatcagcactggcttcctaccagctgggagcagccaggaggatggcttcttctcacctccatctccaggggtgaagatggcattgcttccctgtagtctgtgcgagggactgacaccctgactaggagggactccatcttggggtttaatctcaatcccttcttttttttgtgagatggagtctcactctgtcacccaggctgga

SEQ ID NO: 16303 - RNA, 529 nt, Homo sapiens
  source 1..529: mol_type = other RNA
ggcttgcatgggggactgggcccgcacacgcccccggagcggtagccgaagctgcgtccgcaggagccggcccgaaagcctccgcacacgctgtggctgccgaagcccccggtgaggccgcggtagcaggagatgccacggtagggggcggcggtgatgcagcagcggccgggccggggcccgcaggccgagatgcagctgaaggcgcggccaccacagtaagatccacaagtcatggtgctttttggggaagagaggaggttctgaggatggagacgtccgaatggagagcacagtggtcggggcgtcaggcgttcactacttgcacctctgtaggcctgactctcagcactgcccacctccaccgtcagccactggatggcctgattaagcctgttcagatcctccttgctgggcttcaggctctgcgtgtgtttctgcacagttgcctttaattcctcacactgtggagcagacggcagaggggagctgtagtcaggaggtgaggaggccagacagggctgcccat

SEQ ID NO: 16304 - RNA, 71 nt, Homo sapiens
  source 1..71: mol_type = other RNA
ggctttctagtctcagctctcctccagctcagctggtcaggagagctgagactagaaagcccagggcaggt

SEQ ID NO: 16305 - RNA, 73 nt, Homo sapiens
  source 1..73: mol_type = other RNA
ggctttctagtctcagctctcctgaccagctgagctggaggagagctgagactagaaagcccagggcaggtcc

SEQ ID NO: 16306 - RNA, 3514 nt, Homo sapiens
  source 1..3514: mol_type = other RNA
gggaaaaggaagggggaggagacctgagctaccttaaaccctttgataaccaggccacgtgactcagggcaaccttccgttgctgttttgttaatttatttaaaataggatgactcagtaaaacattttagatgtaagtctcaaagaactgaacttctccattcaggacctgggggaagagcaggtcttaactgaaaagtcgggtgccaaggagccagggagcatctgtttcttcctgataactccccttccactgagaaactgagacagtcaacgaaagtgctccttccagaagcagccccgcctctgtgtgtggcatttcaactacaacgcatccgccaggaaaatgctccagttgatttccattcagggctggataactttatgaccgctaattatatctgcagccacacatggagataggcataaaaatagccttttgtcctttcattaaaggaacctcttcaaatattaacttagcaatctcctccacaaccccccagaggtagtaggcgggtagcaaagttttcatattctgattttacagagtaagatactggggatgcaggggaggctggtgctgtggctttctccaggccaagactataccttcaaacaccaagtggctgataaagactggtgttcttgaagtcaccccttttattccacaagacagaccccaagttttgagggcacggtctatgtgtaaggcctcgggtcctagaaagacgagtgacggacatggtgttagagcccaatacatatttcctgttgtggaaaatgtcttatccatgcacccctctaagtgacataaacacaagacgtttgtcgtacgtgtaagcctaaggatgaaaacaggaaagacacagagtggggtgaaccttgctcacagcagagaaggaaaccagtggcgtggctaaaatactccccctccacagggaatgctcccaacacagaggaagacagacatttgagataacggatatgcttacaagaaaaaagacccccttcatagcacagagaattgggctcaacttgtgcccaacttgtgcccttgcctcttagtgccactatgagccaagtaaaggcatcttcacattcagtcttcatttcctccacatgaaatggagatgaatgcctattctacagcacaagtgtgatgaatgaagacgggaagtcatgcaaaacgctcagcacgggcccctgctcaggcgagcactcaagagaagaagtcaactgaagcctcacagtaagaacctccacggtttcttgtggtcaacaagggaaaacattttggtccccaaaaagaaacaatcctttgtcagtcctattccgtgattatgctcttttaaagcagacacagacaaagccaggagtgatgccccttaaaaatttaactatatatcatattcatttattatcaatccacaggaaaatctgattgctacatgagctcataaaagcttttttcacctttacaaaattaaaaaaaaaaatgtgccacaaggatgtaataacaactgctgataaacaagaaaaggaatcttaaaattataaatttgctgtagaaaagataaaaaacaattatattttatttagaattttaccttgaataaaatattcccctgtataaaaaataaaaaagcttgctctggttagaattagagtatttttgtcttcaaatctgggaatttgcataatatttccatgatactttttcctttgtaccgcgtggcattcaagcatagcagattagaaggattttttttaaagcagtctgaaaatgggacatctgtagagaaattcatttccttcttctcctccggatgtggaatggaagctttgagggaaggaaaagtaggaaaagagcgggatgggatgggatgggatgggatgggatgggatgggataggaagagaggctggggaatgggcagagaagggggtgctgagtgtgctgtgagatagagcaagatcacaagaaggcctatctgtaagtgctttaagataaggtgcagaagcagactgcaatgtcgctagtgctgcctatgtacatattcacaagaataaaaaattccagctagttcacattatctcgtccgttctgaggcatccactccaccttgctggccttgaccgcaggcaatgcagcacctccactgcccttgttggtccttgaacttgagtgagtagccctgggagatccagcaggctctagaaacacacgtctaccaatgggctggagtcctgagttaaagagaagctccagtactggagttggacacagcaatcaatgttctattgtcaaggctttttcccttagatttgtctaaaataggtgtcagagagaaaaaaataaaatacaaacaaacaacaaaacaaagccaagaagccccaacaaccaccgcggagagtcagaggcttaacagctcttgacgcgggcctgggtgatatccgatgttttcttgatgacgctggcccgggtctcccggtctggccgactgctgctggatgctggggtcatggaggaagaaagggggaggtcttgaaaagggggccaggagctgttgtaaggcaccggattgctctcctctttgatggtgacctggaggtccggtttgttggaagtgacgaaggacgccatgccgggcagcaggtaggagcctcgagtccccatgttgctgaggtactgtttgccttcaatattcctcttccgccagtgtggccgcccctcggcactctcttcatcgctgggcacactatcagtcgtttcgctttctgcataggaagacacgggggagatctgcagagggtagagctcgctcatgctgaccggctgctcgtcgctctcagtggtcacctctacaacttggcaaatgtctggcggattggtgacaatctcttgattctcaatgttgctgtccagatgggactgtcctacaactttcttagaaggccgttctgataggggcagcattcggtagaccctgaaggcattatttcctttctttatgcttttatccttgacttcttcaatatcaggcaaggaattcatggcgcatctgaaattcgccttccatgttttgggatcaggtttatctactcctggttgatgctttcctgtatggattgcccagtttctaaagagtggtgcatctttttccacatcccacccatgtctagccgcatgcatccaggggatctgaaaaatcttcttttccttgttaagccacttgagccccgggatcgtgttggagtttatctgctcctccagccacgggcgcatgcgcatcctttccaccggcatggtgccctctcagtgtgcttttttcacgctaccaatacaattccgcaaggtataagtgttgctagggtatgtgaaatggaaatgaaagcccgtcagttgaataatcgcaggagcaaaactaaaagttactccccggcttgcctgagaacagtccagatcgaaagcaaaacaaggagaggaaactgcgaagagccgcggctggaaatcc

SEQ ID NO: 16307 - RNA, 3645 nt, Homo sapiens
  source 1..3645: mol_type = other RNA
gggaaaaggaagggggaggagacctgagctaccttaaaccctttgataaccaggccacgtgactcagggcaaccttccgttgctgttttgttaatttatttaaaataggatgactcagtaaaacattttagatgtaagtctcaaagaactgaacttctccattcaggacctgggggaagagcaggtcttaactgaaaagtcgggtgccaaggagccagggagcatctgtttcttcctgataactccccttccactgagaaactgagacagtcaacgaaagtgctccttccagaagcagccccgcctctgtgtgtggcatttcaactacaacgcatccgccaggaaaatgctccagttgatttccattcagggctggataactttatgaccgctaattatatctgcagccacacatggagataggcataaaaatagccttttgtcctttcattaaaggaacctcttcaaatattaacttagcaatctcctccacaaccccccagaggtagtaggcgggtagcaaagttttcatattctgattttacagagtaagatactggggatgcaggggaggctggtgctgtggctttctccaggccaagactataccttcaaacaccaagtggctgataaagactggtgttcttgaagtcaccccttttattccacaagacagaccccaagttttgagggcacggtctatgtgtaaggcctcgggtcctagaaagacgagtgacggacatggtgttagagcccaatacatatttcctgttgtggaaaatgtcttatccatgcacccctctaagtgacataaacacaagacgtttgtcgtacgtgtaagcctaaggatgaaaacaggaaagacacagagtggggtgaaccttgctcacagcagagaaggaaaccagtggcgtggctaaaatactccccctccacagggaatgctcccaacacagaggaagacagacatttgagataacggatatgcttacaagaaaaaagacccccttcatagcacagagaattgggctcaacttgtgcccaacttgtgcccttgcctcttagtgccactatgagccaagtaaaggcatcttcacattcagtcttcatttcctccacatgaaatggagatgaatgcctattctacagcacaagtgtgatgaatgaagacgggaagtcatgcaaaacgctcagcacgggcccctgctcaggcgagcactcaagagaagaagtcaactgaagcctcacagtaagaacctccacggtttcttgtggtcaacaagggaaaacattttggtccccaaaaagaaacaatcctttgtcagtcctattccgtgattatgctcttttaaagcagacacagacaaagccaggagtgatgccccttaaaaatttaactatatatcatattcatttattatcaatccacaggaaaatctgattgctacatgagctcataaaagcttttttcacctttacaaaattaaaaaaaaaaatgtgccacaaggatgtaataacaactgctgataaacaagaaaaggaatcttaaaattataaatttgctgtagaaaagataaaaaacaattatattttatttagaattttaccttgaataaaatattcccctgtataaaaaataaaaaagcttgctctggttagaattagagtatttttgtcttcaaatctgggaatttgcataatatttccatgatactttttcctttgtaccgcgtggcattcaagcatagcagattagaaggattttttttaaagcagtctgaaaatgggacatctgtagagaaattcatttccttcttctcctccggatgtggaatggaagctttgagggaaggaaaagtaggaaaagagcgggatgggatgggatgggatgggatgggatgggatgggataggaagagaggctggggaatgggcagagaagggggtgctgagtgtgctgtgagatagagcaagatcacaagaaggcctatctgtaagtgctttaagataaggtgcagaagcagactgcaatgtcgctagtgctgcctatgtacatattcacaagaataaaaaattccagctagttcacattatctcgtccgttctgaggcatccactccaccttgctggccttgaccgcaggcaatgcagcacctccactgcccttgttggtccttgaacttgagtgagtagccctgggagatccagcaggctctagaaacacacgtctaccaatgggctggagtcctgagttaaagagaagctccagtactggagttggacacagcaatcaatgttctattgtcaaggctttttcccttagatttgtctaaaataggtgtcagagagaaaaaaataaaatacaaacaaacaacaaaacaaagccaagaagccccaacaaccaccgcggagagtcagaggcttaacagctcttgacgcgggcctgggtgatatccgatgttttcttgatgacgctggcccgggtctcccggtctggccgactgctgctggatgctggggtcatggaggaagaaagggggaggtcttgaaaagggggccaggagctgttgtaaggcaccggattgctctcctctttgatggtgacctggaggtccggtttgttggaagtgacgaaggacgccatgccgggcagcaggtaggagcctcgagtccccatgttgctgaggtactgtttgccttcaatattcctcttccgccagtgtggccgcccctcggcactctcttcatcgctgggcacactatcagtcgtttcgctttctgcataggaagacacgggggagatctgcagagggtagagctcgctcatgctgaccggctgctcgtcgctctcagtggtcacctctacaacttggcaaatgtctggcggattggtgacaatctcttgattctcaatgttgctgtccagatgggactgtcctatgatgttcaccgtactatccacttcattttttatagttgaagtcaggaccgcatactcaggagaaagatcacttactccattactaagccccagagatgactcaactggttcttgcttgatgtgcttaactttgtcttctttttctgtctttggtttctttcctttcttagaaggccgttctgataggggcagcattcggtagaccctgaaggcattatttcctttctttatgcttttatccttgacttcttcaatatcaggcaaggaattcatggcgcatctgaaattcgccttccatgttttgggatcaggtttatctactcctggttgatgctttcctgtatggattgcccagtttctaaagagtggtgcatctttttccacatcccacccatgtctagccgcatgcatccaggggatctgaaaaatcttcttttccttgttaagccacttgagccccgggatcgtgttggagtttatctgctcctccagccacgggcgcatgcgcatcctttccaccggcatggtgccctctcagtgtgcttttttcacgctaccaatacaattccgcaaggtataagtgttgctagggtatgtgaaatggaaatgaaagcccgtcagttgaataatcgcaggagcaaaactaaaagttactccccggcttgcctgagaacagtccagatcgaaagcaaaacaaggagagga

SEQ ID NO: 16308 - RNA, 5015 nt, Homo sapiens
  source 1..5015: mol_type = other RNA
gggaaaaggaagggggaggagacctgagctaccttaaaccctttgataaccaggccacgtgactcagggcaaccttccgttgctgttttgttaatttatttaaaataggatgactcagtaaaacattttagatgtaagtctcaaagaactgaacttctccattcaggacctgggggaagagcaggtcttaactgaaaagtcgggtgccaaggagccagggagcatctgtttcttcctgataactccccttccactgagaaactgagacagtcaacgaaagtgctccttccagaagcagccccgcctctgtgtgtggcatttcaactacaacgcatccgccaggaaaatgctccagttgatttccattcagggctggataactttatgaccgctaattatatctgcagccacacatggagataggcataaaaatagccttttgtcctttcattaaaggaacctcttcaaatattaacttagcaatctcctccacaaccccccagaggtagtaggcgggtagcaaagttttcatattctgattttacagagtaagatactggggatgcaggggaggctggtgctgtggctttctccaggccaagactataccttcaaacaccaagtggctgataaagactggtgttcttgaagtcaccccttttattccacaagacagaccccaagttttgagggcacggtctatgtgtaaggcctcgggtcctagaaagacgagtgacggacatggtgttagagcccaatacatatttcctgttgtggaaaatgtcttatccatgcacccctctaagtgacataaacacaagacgtttgtcgtacgtgtaagcctaaggatgaaaacaggaaagacacagagtggggtgaaccttgctcacagcagagaaggaaaccagtggcgtggctaaaatactccccctccacagggaatgctcccaacacagaggaagacagacatttgagataacggatatgcttacaagaaaaaagacccccttcatagcacagagaattgggctcaacttgtgcccaacttgtgcccttgcctcttagtgccactatgagccaagtaaaggcatcttcacattcagtcttcatttcctccacatgaaatggagatgaatgcctattctacagcacaagtgtgatgaatgaagacgggaagtcatgcaaaacgctcagcacgggcccctgctcaggcgagcactcaagagaagaagtcaactgaagcctcacagtaagaacctccacggtttcttgtggtcaacaagggaaaacattttggtccccaaaaagaaacaatcctttgtcagtcctattccgtgattatgctcttttaaagcagacacagacaaagccaggagtgatgccccttaaaaatttaactatatatcatattcatttattatcaatccacaggaaaatctgattgctacatgagctcataaaagcttttttcacctttacaaaattaaaaaaaaaaatgtgccacaaggatgtaataacaactgctgataaacaagaaaaggaatcttaaaattataaatttgctgtagaaaagataaaaaacaattatattttatttagaattttaccttgaataaaatattcccctgtataaaaaataaaaaagcttgctctggttagaattagagtatttttgtcttcaaatctgggaatttgcataatatttccatgatactttttcctttgtaccgcgtggcattcaagcatagcagattagaaggattttttttaaagcagtctgaaaatgggacatctgtagagaaattcatttccttcttctcctccggatgtggaatggaagctttgagggaaggaaaagtaggaaaagagcgggatgggatgggatgggatgggatgggatgggatgggataggaagagaggctggggaatgggcagagaagggggtgctgagtgtgctgtgagatagagcaagatcacaagaaggcctatctgtaagtgctttaagataaggtgcagaagcagactgcaatgtcgctagtgctgcctatgtacatattcacaagaataaaaaattccagctagttcacattatctcgtccgttctgaggcatccactccaccttgctggccttgaccgcaggcaatgcagcacctccactgcccttgttggtccttgaacttgagtgagtagccctgggagatccagcaggctctagaaacacacgtctaccaatgggctggagtcctgagttaaagagaagctccagtactggagttggacacagcaatcaatgttctattgtcaaggctttttcccttagatttgtctaaaataggtgtcagagagaaaaaaataaaatacaaacaaacaacaaaacaaagccaagaagccccaacaaccaccgcggagagtcagaggcttaacagctcttgacgcgggcctgggtgatatccgatgttttcttgatgacgctggcccgggtctcccggtctggccgactgctgctggatgctggggtcatggaggaagaaagggggaggtcttgaaaagggggccaggagctgttgtaaggcaccggattgctctcctctttgatggtgacctggaggtccggtttgttggaagtgacgaaggacgccatgccgggcagcaggtaggagcctcgagtccccatgttgctgaggtactgtttgccttcaatattcctcttccgccagtgtggccgcccctcggcactctcttcatcgctgggcacactatcagtcgtttcgctttctgcataggaagacacgggggagatctgcagagggtagagctcgctcatgctgaccggctgctcgtcgctctcagtggtcacctctacaacttggcaaatgtctggcggattggtgacaatctcttgattctcaatgttgctgtccagatgggactgtcctatgatgttcaccgtactatccacttcattttttatagttgaagtcaggaccgcatactcaggagaaagatcacttactccattactaagccccagagatgactcaactggttcttgcttgatgtgcttaactttgtcttctttttctgtctttggtttctttcctttcttagaaggccgttctgataggggcagcattcggtagaccctgaaggcattatttcctttctttatgcttttatccttgacttcttcaatatcaggcaaggaattcatggcgcatctgaaattcgccttccatgttttgggatcaggtttatctactcctggttgatgctttcctgtatggattgcccagtttctaaagagtggtgcatctttttccacatcccacccatgtctagccgcatgcatccaggggatctgaaaaatcttcttttccttgttaagccacttgagccccgggatcgtgttggagtttatctgctcctccagccacgggcgcatgcgcatcctttccaccggcatggtgccctgtaaggatgcaagaagaagaaagtctcaccgccgtgatattcttgtaagaaatgcataaccagaaacgtcaacaagcccaaacggatacacattctctaagaaaattgccttgtcattgtcaaaagtgtcaagttcatggaagtcaaggaataatgaaggaggcagggcaccgaaattcaacacctagccctgcatcagattctcctgctgcaagggacatgactgagacattccaacaggaacagggtctgcgggtgggaggcgactcacacagcggtgctagtttcctgattctgatggccgtgccagggtctcaatggagactatcttcgttacagcaaagacacattcaagtactcaggagtgatgggatatcagtattggcaagttactctccaaagatgtagaaaaataattctttgtactattgttaaactgtggtggaagtctgaaattagctcaaaagaaaacgacttggccagaaagacaataccaagtaggtaagtaatttccagtacagagggaaagacgacgacagcctttctgcaaatacaacaaactctaggaaaccccctttgtggtgcttaaatgaagctgctggcggtttattcgtcctccgtgcaccaggatggtattaataagcacatgcatcaatcactttatctatccatccataaggggcagcttaatcaagcaacaattagctgaacaaggaggctctaagcttcatttcctgggggagatgaggagtgatggtccataattcatttaaattgttcagttgtgtagaagaggagaaataagacggccaaagagctctcgtgcgtatttgagagaaaagcgctcagatttaggcgccaaagatttacctccagccaaacttctgtgctaattcaatagaagttatttatgttttatattttaaagcacagaattggtttccaagtcactctgcctcacctcaaagttaaggtggaagaaaaaccgccagaagtgccatcgctgggtcactgatagatttgcaaattgtagatgtttgtcctccagaggcccctccaccaccagttctctgcaggacacttcagggttcccagcgccccaaatctggcattcccagaatagtttcattttcgatcatgacaacagttcccactcccacagcttttcaagcacttggctcagggaagacccactaggagtaagggctttgctttttgtttcttgtttacaacgtttcctcgacgtgtgcaagacggaagcctgaacaactgtcagttccacttgctcgtacttggctgaacactgcagttactcccctggcctcggactccggagaagagcacacagcactgtccaagaacagctcccacactctcagtgtgcttttttcacgctaccaatacaattccgcaaggtataagtgttgctagggtatgtgaaatggaaatgaaagcccgtcagttgaataatcgcaggagcaaaactaaaagttactccccggcttgcctgagaacagtccagatcgaaagcaaaacaaggag

SEQ ID NO: 16309 - RNA, 1710 nt, Homo sapiens
  source 1..1710: mol_type = other RNA
gggaaaaggaagggggaggaggaggaggaggaagaggggaggaggaagagggggaagaagaaggggaggagtaagagggggaggaggaggaagagggggaggaagaggggaggaggaagagtgggatgaagagggggaggaagagggggaggaggaggaagagagggaggaggaggaagaagagggggagggagagggcgaggaggaagagggggagaaggaggaggagggggagaaggaggaggtggaggaggaggaagggggtgaggagcaggaggaggaggagacaaccagataggcatggggatggttccgtctgctcgggctcacttgtccactggcctggatccctcaggcctccatccttccatttcacagcctcagttcctctctggtggggcctccttgggtccccatgaagagactgctctccacgaacctttccttctctgcctgtctggccttccacttctccttttctcttgcccctcaatgcctccgttcccttctctcccacggtgcccagcaagccttcgttacctgcccactctgtccctggccctgtgcctggccccagggtccagaaccccttagcatgatggcagttttttgccctggaggagctcataggctgctgagaagacagacacaaaagaaaataccaagaggccagagagctcactctgcctgggtctcatgcccttatgagggtggtttctgcctggggtaaaccctatgtgttcgaacacctgctgctccactgggccctcagagtggagcacagaccctgcctcgcccccacctcagggagctcagagccatcagaagactgccctgcaggggtggggtggctaccacttactgcttccggctgcaaggagcaggaaacccctacttgaggaacgaaataataataacagtgtgacagctcacatgaagccagaggcaggtggctccagggccggcgagtgcagcaggtccgggatgtcacccaggacgcaggttccttctgtgtttcctcctgctgccctcagcatttcaggttgtcctccagccagctcccctcagggccacaggatggctgccactgctcccatgctgattcccagggctcgtcccagacctggatccaaagccctgaggtgcagggccccagtctccctgggtgcccccaaggtcctggccgctgtttgggagccagtcccccggccttcctgcgtggatacgggaatgctcagccttgagccgggggcacatcagaggagcagtgagggcagcacgtcctggagtgagcagaggctgcagacagggcttccacgcagaccgtttgcctgttaccaaatttgaggacaaaggtttctttcttttgaagtcatgggttcttggatggagccttgtctgaccccagcagtgcagcacaggggagtgaatgagcaggaagacgaccagcatctcctcagggcagggccatgactggggcctgtgcgtccatccccgcggagctggtggcagagtggcggatgccgtggtggagcactgcatggagcactgacggatgacacgtgcacatggcgatgaggacgacacctccttcctgccgtgcccttagttaacttgtccgaggcttggatttctttcttctgcctccctcagaagcctgggctgcacagcttgggctgctagctggcgcggggccacgcgcctgtctgt

SEQ ID NO: 16310 - RNA, 3393 nt, Homo sapiens
  source 1..3393: mol_type = other RNA
gggaaaaggaagggggaggagtggggcttgtaccctgctacaaacctctaggctaggaaatgccaagattgtgtgtaactaagtctaggtgaaaaacttaatcccttaagtcccaaatacccaacttagagaggtacaggaaacggctggtcagcaacatcactccagtgttttaaaaactcagagtacataaacttgagcttattttgcctgttttaggaaataaagaaatataatggcacatagggatttgaaagaatcacaaacacatcagagagatcttatgttaggctgatttataagtgctgctttgggcagttacacagtttgtttacaatgaggagttatttgactttgaacatactgtacatggcaattagaagttgtcatggcaaaagaaaaccacagctggcctgccacagccaacacaagaaccagaaaatggtagatgaaatgaaggaataaaggtggggtttattccttattataaaagaaaaaaaataattcttcagcagtcttaacaaagacatcaagatacaaaattacaagtgttttgactccagccctgtccccatctcctccaagagcagaggtaggagacagttgaagcaaacaagcaattctgtaaaaattacctagaaaccctacaaatttgattaaaatctaaacttctataattttgctttttaaaaaatttaatatcaaaaggcctgctttagtgacatgctattcctaccagaaaataaccccaataccccctctgtcagtaacatgctcaagttgaccagccaactcttatctctaaacctatgtggacaagtgtgtcttttaaaccaaagccacggagatcaagtgactgctagtaacgtgttgtctgttaactaatccagtgcccaccttctccagagggtgggcagggcagaaacccaaaagggtcttgagggcctaatcccagatcaccatctaagaaccacttcccttgctctctactcaaaatgagatgctttatttctaatccgactatttgtctcaaatttggtgccccgtgacctggatggttttttcctttagcaaaacacacataatccacaaaaccatacatatagttttttgtctttacatttaaatataaaaatactattctgctttgtgtgataaatcaaggaccaagcagtaagaaccttttcttctttcaaggtagggatatccatcagtttatactaagcttcgtgttcagagcagggcatttagtcccaagccaggctagtcccacaagcaagagaccaaagccattctctctgattcccaacccctaccttctctcctaattcccacttttaatagaaaagttggttataactttttaagaaaagtttccaccacgagggcaagtcctaacctaaccagagtacgtcaggtcttcccctttcagctacctggaagaagagacccccttctgcaaacgtgctctgtccggatagctacgcctattggacaggtgcaccccattaaatggaagcagtggttatgtctccccaccctcctccccactaatgcactaaaaagcttcagtgatagggaaaaaaaggagggtaggtgtgaagaaattaataacttgacccctctatcccagccaaacaaagaaagcaagattaactgggcacatggaatgaaaaaaacgaccttgatattccaccctttgagttacaatcgggacaactgggagagggggaagagttggagtgggatgaagaactaggaggggctcaacagctggaggtctagtccacttaatttttgtactggaagggctcatcgccggtttcattgagaagacacgtgcggatgagggcttctgtcaccgaaaaggggtcgcagttggcagaggggcgacgatcttcaaagtaacccttcttctcctggccaacagtccggggaatgcgtatgctggcgctacgattggctacaccagcagaaaagtcgttgatgttggaggtttcatggaatccagttagacgtcgggcattgtccaggcctcccttgggatcataggcacggatgtggtactggtgccgcttgcttagtttctcaatggcctcctcgatgtacttcagaccattctcctcccgcatggccttggtgctgaagttggtatggcagcctgcaccattccagttcccaggaatgggcttaggatcaaaggttgctatcactccaaagtcttcacacacacgatgcaagatgaaacgggccacccagagatgatctcccatgctgattccttcacaaggtccaatctgaaattcccactgggcaggcatgacctcggcattagtccccgcaatcttgactccagcatacaagcaggcccggtaatgggcctccacgatgtccctgccataggctctgtctgctcccacaccacagtaatatggaccctggggccctgggaagccgttggaaggccaaccaaaggggtgcccatctgtccccatgagggtatactcctgctccatgccaaaccaggggtgctggttgctcaccatgtccattatccgtttacaggtgtgcctcaaattggtctctgcaggccttcgattgtacttgaaaacttcacataacaccagcttgttagggtccttacggaaggggtcccgaaacatggcagcaggcacgagatacatgtcactgttggaaccctcagactgtaaagtactagagccatcgaaattccactcaggcaactcttccacacacttgggctcactgtccagggtccgggtcttgcagcgcagtccttctccagtaccatcgatccagatatacatggcctggactttctcaccctgaggcagggacatgtacacctgcttgatgcctttatttaagtgggaacttgctgaggtggtcatggtggaaggtgttcccagccacagaaagtcaagcgtatcgttagggttgccctctttaacccttctctttttggagtggcgttcgcgcctctcctctttctcagactctagctggtccaagcaccggagctttctgggagagggcgatggagaaggggacagacagcggccggcccggggggtgtccgaacaggcaggttggtgggttaaggtcttaatcttgactcgagatctctccccggagttcacagagtaggcgacgaagccgaagcagctggagcgcgacccggaggagtctgacttctcgttgtcttcataattttcattcgttgctttcttcgtggacttgcggctgggggaggatccccgctggtcgccgagcaggcgggcgggtaaagctaggccgcgagagcgaggttaggagaggagaggaggccgcagtactgctcacacgctccgctcttctcccactctcgactct

SEQ ID NO: 16311 - RNA, 3092 nt, Homo sapiens
  source 1..3092: mol_type = other RNA
gggaaaaggaagggggaggagtggggcttgtaccctgctacaaacctctaggctaggaaatgccaagattgtgtgtaactaagtctaggtgaaaaacttaatcccttaagtcccaaatacccaacttagagaggtacaggaaacggctggtcagcaacatcactccagtgttttaaaaactcagagtacataaacttgagcttattttgcctgttttaggaaataaagaaatataatggcacatagggatttgaaagaatcacaaacacatcagagagatcttatgttaggctgatttataagtgctgctttgggcagttacacagtttgtttacaatgaggagttatttgactttgaacatactgtacatggcaattagaagttgtcatggcaaaagaaaaccacagctggcctgccacagccaacacaagaaccagaaaatggtagatgaaatgaaggaataaaggtggggtttattccttattataaaagaaaaaaaataattcttcagcagtcttaacaaagacatcaagatacaaaattacaagtgttttgactccagccctgtccccatctcctccaagagcagaggtaggagacagttgaagcaaacaagcaattctgtaaaaattacctagaaaccctacaaatttgattaaaatctaaacttctataattttgctttttaaaaaatttaatatcaaaaggcctgctttagtgacatgctattcctaccagaaaataaccccaataccccctctgtcagtaacatgctcaagttgaccagccaactcttatctctaaacctatgtggacaagtgtgtcttttaaaccaaagccacggagatcaagtgactgctagtaacgtgttgtctgttaactaatccagtgcccaccttctccagagggtgggcagggcagaaacccaaaagggtcttgagggcctaatcccagatcaccatctaagaaccacttcccttgctctctactcaaaatgagatgctttatttctaatccgactatttgtctcaaatttggtgccccgtgacctggatggttttttcctttagcaaaacacacataatccacaaaaccatacatatagttttttgtctttacatttaaatataaaaatactattctgctttgtgtgataaatcaaggaccaagcagtaagaaccttttcttctttcaaggtagggatatccatcagtttatactaagcttcgtgttcagagcagggcatttagtcccaagccaggctagtcccacaagcaagagaccaaagccattctctctgattcccaacccctaccttctctcctaattcccacttttaatagaaaagttggttataactttttaagaaaagtttccaccacgagggcaagtcctaacctaaccagagtacgtcaggtcttcccctttcagctacctggaagaagagacccccttctgcaaacgtgctctgtccggatagctacgcctattggacaggtgcaccccattaaatggaagcagtggttatgtctccccaccctcctccccactaatgcactaaaaagcttcagtgatagggaaaaaaaggagggtaggtgtgaagaaattaataacttgacccctctatcccagccaaacaaagaaagcaagattaactgggcacatggaatgaaaaaaacgaccttgatattccaccctttgagttacaatcgggacaactgggagagggggaagagttggagtgggatgaagaactaggaggggctcaacagctggaggtctagtccacttaatttttgtactggaagggctcatcgccggtttcattgagaagacacgtgcggatgagggcttctgtcaccgaaaaggggtcgcagttggcagaggggcgacgatcttcaaagtaacccttcttctcctggccaacagtccggggaatgcgtatgctggcgctacgattggctacaccagcagaaaagtcgttgatgttggaggtttcatggaatccagttagacgtcgggcattgtccaggcctcccttgggatcataggcacggatgtggtactggtgccgcttgcttagtttctcaatggcctcctcgatgtacttcagaccattctcctcccgcatggccttggtgctgaagttggtatggcagcctgcaccattccagttcccaggaatgggcttaggatcaaaggttgctatcactccaaagtcttcacacacacgatgcaagatgaaacgggccacccagagatgatctcccatgctgattccttcacaaggtccaatctgaaattcccactgggcaggcatgacctcggcattagtccccgcaatcttgactccagcatacaagcaggcccggtaatgggcctccacgatgtccctgccataggctctgtctgctcccacaccacagtaatatggaccctggggccctgggaagccgttggaaggccaaccaaaggggtgcccatctgtccccatgagggtatactcctgctccatgccaaaccaggggtgctggttgctcaccatgtccattatccgtttacaggtgtgcctcaaattggtctctgcaggccttcgattgtacttgaaaacttcacataacaccagcttgttagggtccttacggaaggggtcccgaaacatggcagcaggcacgagatacatgtcactgttggaaccctcagactgtaaagtactagagccatcgaaattccactcaggcaactcttccacacacttgggctcactgtccagggtccgggtcttgcagcgcagtccttctccagtaccatcgatccagatatacatggcctggactttctcaccctgaggcagggacatgtacacctgcttgatgcctttatttaagtgggaacttgctgaggtggtcatggtggaaggtgttcgttacacgccgcaatcgaggcgtctcaaccatcgccagaaccaggacgattgctccgaaggccccaccacgaggaaggcagccaggcgcccgcgccaaccaagcgccttgtttgcgctccacaggggaccgcaccgccactccatccacagcgcaaacaaaccact

SEQ ID NO: 16312 - RNA, 3037 nt, Homo sapiens
  source 1..3037: mol_type = other RNA
gggaaaaggaagggggaggagtggggcttgtaccctgctacaaacctctaggctaggaaatgccaagattgtgtgtaactaagtctaggtgaaaaacttaatcccttaagtcccaaatacccaacttagagaggtacaggaaacggctggtcagcaacatcactccagtgttttaaaaactcagagtacataaacttgagcttattttgcctgttttaggaaataaagaaatataatggcacatagggatttgaaagaatcacaaacacatcagagagatcttatgttaggctgatttataagtgctgctttgggcagttacacagtttgtttacaatgaggagttatttgactttgaacatactgtacatggcaattagaagttgtcatggcaaaagaaaaccacagctggcctgccacagccaacacaagaaccagaaaatggtagatgaaatgaaggaataaaggtggggtttattccttattataaaagaaaaaaaataattcttcagcagtcttaacaaagacatcaagatacaaaattacaagtgttttgactccagccctgtccccatctcctccaagagcagaggtaggagacagttgaagcaaacaagcaattctgtaaaaattacctagaaaccctacaaatttgattaaaatctaaacttctataattttgctttttaaaaaatttaatatcaaaaggcctgctttagtgacatgctattcctaccagaaaataaccccaataccccctctgtcagtaacatgctcaagttgaccagccaactcttatctctaaacctatgtggacaagtgtgtcttttaaaccaaagccacggagatcaagtgactgctagtaacgtgttgtctgttaactaatccagtgcccaccttctccagagggtgggcagggcagaaacccaaaagggtcttgagggcctaatcccagatcaccatctaagaaccacttcccttgctctctactcaaaatgagatgctttatttctaatccgactatttgtctcaaatttggtgccccgtgacctggatggttttttcctttagcaaaacacacataatccacaaaaccatacatatagttttttgtctttacatttaaatataaaaatactattctgctttgtgtgataaatcaaggaccaagcagtaagaaccttttcttctttcaaggtagggatatccatcagtttatactaagcttcgtgttcagagcagggcatttagtcccaagccaggctagtcccacaagcaagagaccaaagccattctctctgattcccaacccctaccttctctcctaattcccacttttaatagaaaagttggttataactttttaagaaaagtttccaccacgagggcaagtcctaacctaaccagagtacgtcaggtcttcccctttcagctacctggaagaagagacccccttctgcaaacgtgctctgtccggatagctacgcctattggacaggtgcaccccattaaatggaagcagtggttatgtctccccaccctcctccccactaatgcactaaaaagcttcagtgatagggaaaaaaaggagggtaggtgtgaagaaattaataacttgacccctctatcccagccaaacaaagaaagcaagattaactgggcacatggaatgaaaaaaacgaccttgatattccaccctttgagttacaatcgggacaactgggagagggggaagagttggagtgggatgaagaactaggaggggctcaacagctggaggtctagtccacttaatttttgtactggaagggctcatcgccggtttcattgagaagacacgtgcggatgagggcttctgtcaccgaaaaggggtcgcagttggcagaggggcgacgatcttcaaagtaacccttcttctcctggccaacagtccggggaatgcgtatgctggcgctacgattggctacaccagcagaaaagtcgttgatgttggaggtttcatggaatccagttagacgtcgggcattgtccaggcctcccttgggatcataggcacggatgtggtactggtgccgcttgcttagtttctcaatggcctcctcgatgtacttcagaccattctcctcccgcatggccttggtgctgaagttggtatggcagcctgcaccattccagttcccaggaatgggcttaggatcaaaggttgctatcactccaaagtcttcacacacacgatgcaagatgaaacgggccacccagagatgatctcccatgctgattccttcacaaggtccaatctgaaattcccactgggcaggcatgacctcggcattagtccccgcaatcttgactccagcatacaagcaggcccggtaatgggcctccacgatgtccctgccataggctctgtctgctcccacaccacagtaatatggaccctggggccctgggaagccgttggaaggccaaccaaaggggtgcccatctgtccccatgagggtatactcctgctccatgccaaaccaggggtgctggttgctcaccatgtccattatccgtttacaggtgtgcctcaaattggtctctgcaggccttcgattgtacttgaaaacttcacataacaccagcttgttagggtccttacggaaggggtcccgaaacatggcagcaggcacgagatacatgtcactgttggaaccctcagactgtaaagtactagagccatcgaaattccactcaggcaactcttccacacacttgggctcactgtccagggtccgggtcttgcagcgcagtccttctccagtaccatcgatccagatatacatggcctggactttctcaccctgaggcagggacatgtacacctgcttgatgcctttatttaagtgggaacttgctgaggtggtcatggtggaaggtgttctggtcgccgagcaggcgggcgggtaaagctaggccgcgagagcgaggttaggagaggagaggaggccgcagtactgctcacacgctccgctcttctcccactctcgactct

SEQ ID NO: 16313 - RNA, 125 nt, Homo sapiens
  source 1..125: mol_type = other RNA
gggaccatcctgcctgctgtggctcgctcgcctgctccccactcaccctctgaccggctcctagcagcctccactataagcggacgactcctgctcagtcggcctccctaccccagcctcgctct

SEQ ID NO: 16314 - RNA, 3624 nt, Homo sapiens
  source 1..3624: mol_type = other RNA
gggaccatcctgcctgctgtgggcctgcgtgctgtccaaacagcctgggcacccgagattgtctcgccggccaatcacagcaagtgtggagcccgcggccgttccctgcgcacagtagtccctgcctcgtgcccaccgtaaagactgcctttatcactcgggaggttcattcattcatttactattcatttattctttcattcactcagcaaatatttacaaagccctcactccgcgtgaggacagtacagacatgaattaagtacacatggttccacggttcttagtggttccgaccaggagataaggaaatccttgtttgccgtctgtagggctcgctgctctttcttgcttgccagggtgttctggtaacagcaccctgattttcctcagaacagcaccttgctgcttcagtctacaaatctggagggcctggtccagctctagctctgtcgtgagcaggtgaccaggctagaccagatgagcctcacacccctggtgatagccactaagtagtcacaggtgtgggcacatgactctcttcaggccattgaggctcagtcctgggacccttactagaaggactcatgagtccagaaacagtggaagttgcctaggcaaccggttcaggccaaagattgatcttccactagtccaggaagtcttcctggaggtgaaacttcaggtctttaaattatgggagagaagagagtgaagccagcactcacgtgtgaccaccatccacctactgacccattcatccaatgcagtgagggcacatggcacggcatgccgggtgggctgtgtttttactctgtcatatgcttcctgcgttggttccctccagcctgtgcaccccaccctgctccacccctgcttgtgaactaaatgaagatctaagtgatcacatctccacagtgagaaaagacaccaattgtcccagagaaccaaatgcaggaggtgctggtctttataggggacctggggaagacactaactcttctctaaggggtgctccaggctgctctggcagtcgaaagagctagctgcaaggccaaactatgctactgagctgctgtgtgaccttgggcaaacagcttcccttctctgggctacatgatctctaggcatctgtccaataaatacactatttctaaatcaattagacagaaatgctgaggcttggaacaggagccagagaacgtgaggctgaccagtgaccccttaggaaggtggctgccatctgtcctgtttcggaagcctctccctctgctggactccaaaagccctgccttgaaacagctgccctaccactcccaatgcaacttcccaataccatttctctcttttcatttttcttctgttccaaggcagaacagggtaggaaatcgtgtcaaataaagacagaagtgcttgatgttcctaatggcatcccaaggaaatgaagtgtaaaatcacacgagttatttagcttcacatactgcttttatcagagtcctggacagaactccttagcaggagaaagcctgatttccttggaaagatggaattctggtgacagcagcagggagctgggctctcccggcaccgatgcaggatggaaaggtctgtaagtcacgccgaggcaaaaaccaagacacaaatcgccccccaccccaacgcacacacacacacacagagcaagaccacattttatccccacttttcaaaggcaaagttgtgtgtgggctttcactcagccagctttgaaagatcccttaactccaggatgctcttagagtaaaatccgaactccctgctttgtcttccaagcccaacaaagttggagccagccttgggttccagcttaccctgcgcactctccctcctcaaggccctccggtccgcctggctcctttctgttcctcgaagactccaggctcatgccacctaggagcatcgccctgaagtgcgtcttgtccagagtgctcctgcatagctgtcccctccttcccttcagggctcagctcaaatgccatttgttctgagaagcatccctggactacccctggtccgagcaggccactctttttggttttctcctggcatttatcactctctgggattgcattgtttattcgttgtttattttctgattcctcctcctagaaagtgaatggtggggtgggggagaggaagacaggaattacactggttttgttcatcattgtatcctcagagtcctcaacagtgcctagcacaggatgggtaaatctgccggagttcaactggaaaagtggaaataggagttatatacatgtaaattattttatgggatttgttatggagaattggcttatgcatttgtgggaaccgggtaagcagtctttgtcaggctgcgtgtcaagtctgatgctggtgtcaggtccacaggataggcagtcgagaggaaaggcagatgtcaagtagggagagcaagaacccacgagcacaagctagagccccaggatggcagcctgaagcccgtggctattcttgttgcctctgaccacagtggtgaggctgtcctgcagaagcctagcccttcatcacagagctgaacacatacacgcggctgggagtcgaaaagtagcaagaagttgccggggaaggttgcgggtgttgtggcaggctgcttcactccagtgaggtgagtcagcagatcagcagcaacgtgtgtcaactgcaaaacacggctgcagcctctcttgccttctgaatcttgcaagaaccttccaagaatcttccctgtggtccatctgaactgcaaacatgcaggaaagataattccaggaaatgcagttgagcctggccaagttaatagtctctgaagccatcataggtccacatcaacgcatgagctattgatgtgtccaacttgccctgtgacttgttcatctgtgaatgtcctgcacaatttcacagtaccttatttgatcttcacaataaccccagagaagtagacagggcgcggattacgaggattacgaaaaacccacatttttttctttttttcttaacagataagggctctaaaggcttaaagtcactcgagggaggtcagagagtttggggactaaatctcgagtctctcattaattcatgcacatatttaaaaaatatttatccggagcctgttccaagccagatgagatggcagtgggtacaaagatgaataaaacactgtccctgcgtaggaagaagatcacgttctagcctgggggagagcgccaggaaaagtaaacaggtccccccctgctttgtgaggtgatgagtgctggggagataggaagagagtggggaccatgtttctaatctgattctcctaccgacgaccagctcagttgttatttacaaatacctgtcccctaaaggggggagcggggttgggggggcttggccgtgctgctggggtcagagctcgcaggggggttctgccgcagtgtggggacaaactctcccttattgggcaaatatttcccggggcgctacgctaagcacacgggctccccgaatttccctccccagggcctctctgtctttggatggcctgtcagcaagtccctgcagcctccagcccggcccgcgcggcgacccagtcccctg

SEQ ID NO: 16315 - RNA, 961 nt, Homo sapiens
  source 1..961: mol_type = other RNA
gggaggtgtgatctcacactcgttggaggccggacagctgtactcgatgctcccctggatggtcctcttgaagaaggctttgcaggcctcacaggatgccacaccatagtggtagccggaggccacgtccccacagaccaggcagaggcgcttgggcagggagctgagcaccagcttcccaccgccctgctcgccaggcccagccccctccccatcctcctcttccttgtggcctgggaggcagcgagtgggagctggaccaggggccagggccacaggaggctcggtctctgtctccgaggaaccctttggactgtcagggctggccggctctgccttgatgtagagaggctcaatgcccaccacctggctggacatggcgctggtcacctgacacgcggctgccctcctgccccagcatgccggtcccaggcacacggcgggcgccgctccacctcctcgcgaccagcctgcaggtccactcttatactcccgctgtcgcagaggccgccacctcccggggcgccgcgtcccgcccccaacctgcgcacacctttgggaagttgcctaaagttgctacgcctccccctccccgcccgcgggagacctctaccaggttatcaggaagtaagtggggagagccaaggaggaggaagttctcccctgccggtgcgatgacctttgacccagagaggagggtggccccaggccccttcgagcgcccccacgtggtcttcagagccccttcccagacatagagccctccccgtcttccaccccggccagccccagggacttcggcaaatgcgggattgaaccctgccccggagcgggctggatcggaggcccaaccctgacccgagtcaggacccgcagccagagccagatcctgccccaggccggcccaccaggactcggacgccggatcccgcctgaaccctgaccagtccgaccctcgact

SEQ ID NO: 16316 - RNA, 1103 nt, Homo sapiens
  source 1..1103: mol_type = other RNA
gggaggtgtgatctcacactcgttggaggccggacagctgtactcgatgctcccctggatggtcctcttgaagaaggctttgcaggcctcacaggatgccacaccatagtggtagccggaggccacgtccccacagaccaggcagaggcgcttgggcagggagctgagcaccagcttcccaccgccctgctcgccaggcccagccccctccccatcctcctcttccttgtggcctgggaggcagcgagtgggagctggaccaggggccagggccacaggaggctcggtctctgtctccgaggaaccctttggactgtcagggctggccggctctgccttgatgtagagaggctcaatgcccaccacctggctggacatggcgctggtcacctgcacggagagacccataggttcgcaggaaagcactggtatgggggatgggagacaccctgccacacgggttgcccaacctcgggcctagggccaggcttccaagcccagcaagtggggaagaaggggggcagagtccaaggaaggactgcccaggaacactgccccctcctagctgttgccatggaaacagagtcttcagggccagtaactgacagcaggtctcccccttgggaacctgggggaggcttagaaagcccctactcccacccaggccagggagcagggtaaccgtagcccccaggcaaccttcaaccccacctggaatccctagccaggagcaggatacttcccagttttctccagatgttggggggacctctgagaccctgccctcatctgggtattctgcattggagagcagacccaaggccagtggacgtgctcacaccgagttcacacactccactcaccggggtgctcaggagccccacaagcccacgcaggctcgctctctgctgagggctttcacacttgcaccggccttcccaaacccgtgctcactcctgctcacacttgtgctcacacacttctcctggagcgcacaccccatccacgaactcagtcaaggctcatgatcacacacactctcactaggtctccccacatccacacgcacaggcacggactcatgaaaacacctccagagcttt

SEQ ID NO: 16317 - RNA, 603 nt, Homo sapiens
  source 1..603: mol_type = other RNA
gggaggtgtgatctcacactcgttggaggccggacagctgtactcgatgctcccctggatggtcctcttgaagaaggctttgcaggcctcacaggatgccacaccatagtggtagccggaggccacgtccccacagaccaggcagaggcgcttgggcagggagctgagcaccagcttcccaccgccctgctcgccaggcccagccccctccccatcctcctcttccttgtggcctgggaggcagcgagtgggagctggaccaggggccagggccacaggaggctcggtctctgtctccgaggaaccctttggactgtcagggctggccggctctgccttgatgtagagaggctcaatgcccaccacctggctggacatggcgctggtcacctggggctccggcagcgcggtcgggcaggcatgggggccgagcggcccggagtgccggagtgagccgggggccgcgggcggcccctcctccgccgcctcctcgggccgcgccgccccaccgcgccgcgtcccctcactcggcggcgccgccggctgcttgtaggacacaaaaggacatcgcggccgcttcctactccgcttcctccagctgac

SEQ ID NO: 16318 - RNA, 16346 nt, Homo sapiens
  source 1..16346: mol_type = other RNA
gggattctgtagcttcctcctccctgtgactgttataatttctttcttttcttttcttttcttttttttttttttttttttgagatggagtctcactctgtcacccaggctgaagtgcaatggcaccatcttggctcactgcaacctccgcctcctgggttcaagtgattctcctgcctcagcctcctgagtagctgagattacaggcatgtgccatcataccaagctcatttttgtatttttagtagagacgaggttttgccattttggccaggctggtctcgaactcctaatctcaggtgatccacctgcctcagcctccaaaagtgctgggattactaagcatgagccaccgcgcctgacggactgttataatttctgagaaacaatttaacttgtgctccgtgcacaatgctaggccttgttagagatacaggacttaggggcttccttggacccaaacccagaaaagacacgttgtacccttccctaaggctgattgcacacaaggtgaaatggagagcagagcaggacccagatggcccagagtagtagtagaaaagccactggaaccagagccagggacttggcttatggtcctggctctgagactaattaggtctttgggcaacattgctgtgcttctcttggcctcagctttctcatctttaaaatgaaggggctgaactgtaatctctgagagtccactcagcttaaatggaatcgtggtctcttcctacaggaatctagattttttggaaaacctgcctttgggatctagctaggctatgtattagcgttcttaagctattcattctccatatttgtgaaatgatacaaaaaaatcctgcttacctcactgtgttgtcatgaaaactaaaaagagctgaacccatgtgagatctttatgtcattccctcgaagaggtatgtgaatgatagaattaaagtgctagccttccctaagttttgtatgtcttggtatacattgaaggttcttagctaaagggatgagattctgacagtggaattccaagcatcagccagaattgggtgggaaaacctttcctgcattctcatgagctctgcagatagtctttattgtttttaaacccagccgtttaatcagacctcaaggaggcttttctattggagcttacagacttgtccaaactaaaaagaatatctaaacctggaggagggggatgtaggagggagaatgagtaagaaaatgttttgttaatgaataaagatcctgtatttcattcctgaaagctctcactttgctttaggaccatcagcagaagcacagagctagcttaataagctgtaggacgtgaaaaagtcactggtaggtccagggaagttctcagctgaaggggaccctggggaattgtccagtccacccccagccctaccttgcaaccagacaaatgaagctgtctgctagaaaatctggagataccctttcacatttccacaatgacaaagttgtgtgtgggagtccccaggaatcatttataactgaaagaaaaggaaaagccaccttcaaactccagttccaatagacctgagatctttccggaaacccaaaggaactgcctcatttggttttcccagagaatatgaacaacagatcaaactaatccaacctagtggaagaaggatctgtagagtttgggctaatttcttagtaatattcagctgcagccacttcccttctgtttaattttcacgtatcttagtgcttgaattcgtaattcatacccttgttttgaattcccactaccaacagattccataaggccattcatgtcaaacaccctccaaacagttccaagaaaaggactgagctagaattcttttctgaacagtcagaggggctatggacctggtttatatgagtagcatgttctcataacccccaaatccttgacagacattccagggacatggccacttctgccatgtagccaccatttcaatcaggcctcctcaaacaacttactcctaatttctacaatatgtaggtggcaactgtagcccaacgggtgtccgtagatacaaaccaaagctggctaaaaccatgtctggaaagctgacaaatttccaggcaatctaccctgagcagcagacagaaataaaagagctggtaagaagagaaacagacatataatataacagagtttcctgaaattcattataccaaacttccaggatagatcaaggaattggacctaattctgccctgattattttgggtatgtcattatcaatgttgcagaaacatttttaagccactgtctatcaacaatttgatgaaaaaaaaaaaactaacatttcacgagtaatgttgagtgcacagtgattttgaaagaatcactattagtaaactaaacagcactctaaataaagaaaatgactgctgttaagacatactgtctgagaattctcaggaagaacaccacaacgctaactctgctgtatataagaaattattccagtatgcatttgagtaattctgcattttaatttaaccctttgaaacattaatcaaaccatggctaattataggaattaaggaattaaacgatggaatcttctaaaagatattatttaaaaggcagtttatacaattacttgtatagatgtttgctttaaagaggaaaacagttctactgtaatgaaaagggtcttagaaaattaaattaacaaggggggaccaggctgatatgaaactaaattagcatcaaatgcaaattacagggtacttaatggtagaaacaggtgcagagaagaaccctaaatgagataaatgaataaaacatccctctccacaaatgtggaagctgacacaaagtcaatgatatgaataattcagcagcctccacactgctgttgaggtcagcctgccttgacctttgaaacaggaagtaaaattcagttcaaatttgagtgactagaaatataacagtcatttgttttttatattaaaaaatcaacagaattttttaaaaatacaaatacagaaaatataaaatagaattacagtttgaactagagacattatacaatcaaagtacttagtaaacaaacaaaataatttgataagattttacccaaaccatacttcaatatggaaatcctaaaaataaaaataattaaaaacatatataccagtgctcagcttaatgaaactccctgtgagaataaatttttaaatcgttatcctttcttcaaagtattttgttgtgttgctatcaatgtaaaaaaagcatgtcataatttttaaaagccacatattcttattagtaatgcaaaataatttctcatatttgaaagataaaatttggttaaactagatttttaaaaatctatgtaaagttgctattttttaattcttcaattcctgattgaataaatactgcatcctccaaaactattcaccttagaaaaatgcaacctaggttctaaaaacaaactattctcataaccgaatatctattgtggttttacgtgtcttttatcctttttttttctttttgcatgcttcaaaagtattttgtacagtcaaatagtgaaagtactctcctcatttcaaattgaatttagtgctgttagagattaacagggtatgacaacaaaccaatttctacaagctagaaagacagcaaaatatatatggtatatcaccctcgtccttattttacaggatggcataaaagatgtttgataatagcagttatctctgccctccaattggttctattaaggggacccacaacttggctatctacctttcatctatctactgtgcttgtcagataaaagattatgttgaaagatgagcttaattttattttctagatttagagagggttaaagctacatacacacacacacacacacacacacacacacacacacacatacccctcagccatctatgagagagcagtggtaaactaggtctatgattgtaatcactgtaggaagaagtttgagaaatgttccttccaaaccggagtgtttagttgaggcaaaattaaagatgcagggtgtgctgggtatttcttaattattattattattattatcatatctgctaaatcactcctcgctcgacatttaatacagggtgatagacaaaacactgctgatttggggtttgccataatgactgacctgagcaaaggctttgtgtacaaagtggctccccattaaataagggctctgtggaaccagctggttctcattttgaaacaaccggtttctgtatccccaagtgctaaagaaaataatccctgccatctatgactgcacactttcacagaggcagcaacgagaatttgattgtggagataattaaagtcattcctggaacttccaagaaaaaaaaaaaggtggaaagaggtggggtagaaagaaagaatagtcaatgatagtgtttaaaattaaactatgacaaatcattttgagtggagaagagggaggaggagcccccgccctttatggaattcagttgaaacagctctgttttcttccccactcggctgctccagagggaggtccgagatgcgattagtcagggcgacggcccccagtgtccggctcggaagccgaagaatcgaaacatggctcaagaagctacttgtcactgatgacacatcacaatgagattgttttgttttttttttttttacgtttcaatcctaaataaaatagccgcggaggaatctaactggactcttcaacaaacattctttcctagttgatctgaaatgctgaggttagtttaatataatattaagaaaaaaaagagtgtatcagacattcagagacactcatctttcaatcttgaggagagcttattcttttattattttttgaatgctacattgttctacaataagaatccatgttcaaatagcctgaatgacattcagctgaacctacgttccctgcctgcctacattatttcataagcttttgggaaaaaactaaaatatgtgtaatctgtctgtctgcgctatctgcctttaacaggaagaagagatgggctcaatgaggacgactcacggcctctcaattaacctgattagttcagcacattgctctcatgaatgacaccttatcttaaaataagggagaacttccttcctcgagtagacacaggagccccctaaagccacaaagatgcagcctatcaaatgtgagggcctctgcttctcctccctcttcccagctcgcaggtcagagagactagcaggccaggcgcctgattggattttgtgtcctaaggacagaaggcaagctcccgtctgcccaggtggccttggagaaggctggggaaagggatgccctgtgggtaacttcaagccccttctttcagagtcaaccaggcacatgatgggattgggggtgggggacaggaagattggggagggggagggagggaaagagaattcattaacccttcaatctccagagtatcaggtcaatgctatacctgcctgaaagaaaaactggtgaattctgaagtcttctaatagtatataaaacaaaggcgctgcttgcacaggggtctttctaacactgatttcgcgtttgacataatagaggatggctgaatttttgccctgcaaaaatcaagccttctcccaaactctctgaaatctggtggtttgcaaaggatgccacatatatatgtttttacaaaataagaaattcccattatcatgtgtaatacacatagttaatagaatatattcttgaaaatatgctttgtgagaatgtcaacagcagagattttcacttgtctgctctgtgatttacttgatcaattaaacagttaggcaatgaggagatttgcatggtaatcgtgtgaagattaacatttttaagtgtaacaaatttaatattttatcttacattttctgttcctcatcattctttaatggcagtgccatttcactttattgtgtagttataacaagcttgtctttagacagagagatgagaccaccagattcaacaactgcatttctagttcctgtcattccttcttttcacaaaaacaagccctaagcatctagtacacaggagggaggcactgtgctcaacgtagtcactgccctcttaggcttacaacctaccctccaaagcgctcatctacctgcctgtgctcagcaataccacaaacagctaaaattagaattccatagttggaaagggtcttagagatctcttccttcagtcttaaccaacatgtagactgcctcagaagagtgcaataaagccgtggaatttgcccaagttcgatacctctgggtatgagctaaaaggtgactttaacccggggatatttttcttctgcatcatgatcccagtgtaaaatggcattcttctatttttaaaacatatatatcaatatattctttgtttatacttgctattactattccaactatttttgggggactgggggcagagatcaaccctgagacactgagaaagctgcatgaagccaggaactatgtttgtctttttcactgttatacccccaaccctgaaaacagtgcatgacatataatagaggcttaataaatatttgtggaaacaaaacaatgaatgagtctttatctaaggagacttagctaccatgattaacttcagtaaggtaattgtgctcaaaggaagtcccatggcaatgatcacattaagaatgaaaatccacatggaatatacgatgctcaaattgcaagagctacctgattttaagcacctgttatgtgccaagcccagtgctaggtgtttcaatcctcacaacgcttcaaaatagaagtgacttttcccattttgaagatgagaaaactgagccccctgaggctcagctactaataagtagctgtggaggaactggatcccttagccaatgcactccaaaatctatgcctttgccatcatactgtgccttctcccagatttctgtatggattactgatgtttttttcaagcaaatacacaatcaaattaaatgaggacataagaactcaaacattgctccagcaatgagtacaataaacagtgtcacatatgtatatatgcatatatgtgtgtgtatatatatgtgtttatatatatgtgtgtgtatatatacatataaaatcctgaaagttaattgtgacatcaactaagaaagctggcttggtaaataggtttagagtaatacatgaaaatgtgctgtggatagcaagaaaaatgaaataaaagagacattatgaaatactgaaaacagtgtttttagctgagcaattgagaaaagggaaaaaaatcagtctgggagataggagatgtggagtttctaatcacttgctttgtcaccaataaagtggatagttccttaggctgtgtgcctcagtttacagatctgtcaaatggagtcaatttgtgcaaagagaattttctgagatggtataccccgacgtgctctaaaacgctggaagtgccatttaggtgtaagctactattaaactcacagtgatcaggggttttgcttgctttgttttaaggtgctcatagaccaggattcagatgctggtcttcacgagccagatcagggcactcccatttctacagctacaggaagaacaactcagtgtttaaaaccatattctgagacatatcccatatatctaacattagaatctggctttaggaaaacaacaagactgtgtagagaaacatgggttttcaactgttggtaacagcttcaaagataaccaggtgaacccttaaccaactttcttttctaaagaactttttaaaaaatgaaaaagagactgctctcttttcatctttttttttttttttttttttttttggtctctgtagagtatgtgcgtgtgtgtatgtgcgtatgtgtgtggtgtgtgtagctaaacctgatgcaggtccatagttcttcaaattaactttccattctgtgagggggcttcagccaatagtgcacccaagagtgttaaaagtgatattttcagatattactaacagatcagaatacttatgaacgagaagcacattaaaaacaggtggggaaaatctcagtagtttacctctggaaaacaataaataaattgcaagcagcatgactgtctgatattcaggtggagtaataaagagctttagtcaaatcatggttgcttcaggaaggtggaggagggaacaaccttttgaccattagaaaagttacccagctgggctcctgactcctcggcatgcaccagcagagtctaagtcgcgtgcaccacccggcaaaggcggagaattcacggcactggcggggagcagcaccacatcaaaaagcagcagctgatgtcatgaaacaaaataccctatcattttactttgataattttcaattcatcaattaaaaaagaaaagaaaaaaagttatttcagccttgaagatgtcatgtcctgagccccagtgttcacaccctacagaagggctcttcctacccacacatggtatcaatattaagttaattgagcagcaaatgagcaaaaaagttcttgagggattcttgatattgattaaaaggacattaaaaaaaaaacccaccacaacctttacatgaaccaaaatttgagaatgtcgccaaagccccataaaatatgtataatagtgacagtgtccagattaaaaatgtacatgggcagcttgattactattttctggttttttccctgccctggctctgaaagtgttaaagaaaacaataaaagaacaagtgagtgtacagggtaggatttactggcatttacttttaatctatggcccttcactctgtagcttatcgggcctctgtcagtcctttttccccctttatatttcatgaggagccccccatgctgctactgagagacagagcccaagtgtctatgagctttttgtcaggtaaaaagagaagaaaaaggaaaggaacaagaggaaaagcaaagctaagaggcatctattagatgtcactaggcttttgtattcatgtcaatgattcaggattagagtatttgaaataatcttattgagaggaatcaaaaggcccaccgagtgagaggctgctctgtagcatatggcaaaggcacgaacaatatcttattaaagatgtgttggctaacaccattactttatattatattacaaaactattgtgcctcaaacagttagcaggatggtatagttaccaagtgccattttggaggttattgtgtaggatcaatctatataatttgccagcatgtctagctcagtcatgacaagtagggtttagggcatgtttgcaactggaaccaagcacttcactttcaaaaatagaaattcccaaagcacacagaagaccactctgttcccaccgaaagtggagtacacatttcatagatggaacgccaatggcctgtccttccccagaatcagtttaattaagtttgcatcatttaacatatgtgacaccccctgccccacccatgaaaaatgtaacaaagattttttttttttgcatgactcccctccctattaggaatacatgcacagacacacacacacacacacacacactcagcttcacactttagcaggattagggcaattaaaattctattagaataagtactgtaacgttaaaaccttcttttgcttctggacaaagacttgtaactggagaaatagtttgtaagggagatttttcttcctctacccacacctttcaaggcagggagcaatgaaagacaaacctgtactgttcaccatatttcattgattgcaataggagtattgaggtcacttttatattgtcctggatagtatgtagttacgcggtttgtaaagagaggaatgggatggggggctgtgagaaggaagaattagtggtcgatttcagataacatctcatgcaaattaaagtgaccaaaataccatctctttacgcaggaaccactaaatggagttttttaaatctggtcaatttttattagagagttaaccgggtgctggcaggagagggaaatgaggaaatgaggggaatttatcaatggagagttacacttggagagagtttttccccccattctaagcaacttcttttaggaaagtaaaagcatgtttaatatactcatatattctcattacaaaatgattgtgcatagttactaatgggacacacagaggacttcgtactgcttttctgtatttttccagaactgttacaaaagcaaagttatgatgacatgggattaaaaacctacaccacgggctgatacccgggccatgctacacatacacactactgattctctgaagctccgttaaatacatttcttggaagttgctgccattatttcctttacaggaaaaccactgttgttcattatacagtgtctgcaatagtattataccatgtaaaagtactttgcattatgatacattgtcagcgtattcgaaatgcattttaatgcatcctggttgtgtatttgggaatagctgatagcaaatggaatatagactgcgattagcttattgtattagttattttcttatcacggtagcaaactgcacacaaatgtacggggctcatctcatattcagaatggtattatctgatatgtgataaaatttagaatgatactcattcacataagtctcatcgctaataatcacatatgaattcccactgagaagacaaatgtttaaacacactaaggttaataaacagtcttaaattcatgctcagtgtcaatgctggcttttcacttttgaaaaaatgcaaacctctcaaaccaaccaaaaacacaataattatcctgcctagggcaattttagagagtgaattcctcctccttttattttaaccaagcagtcaaggttacaaatcaggtggtataaaaggtttatcggaacgctgagaaatgcatttacacctctggttcttcataccccacacagccatttgtgtatagtgcagaatgattatgcattggtggtggttggtccttctaaaaactggatgaagaccaaaataagaagagttgaaagggcattgaaatgaaatcatgaaactaactaaaagcctcatttgcaactttaataaaattatatatttatgttcatgttaattgaggactttatgtggatgacaaaaaataaataaatattggaatttacctctgattataaaagacagaggaaagccattgattgttgaaaggcccagatgcctttacaatccttggcaaatacataccacacccgacccaatggtaaaaagtatgtgggtgggtggatggatggatggatggatggatggatggatggatggttagatagatagatctctcctaactctaaagtttttatattgttttcctattatacatatgggcatatatgttatataaatacattggtgtcaatttaatgaagaaaattagcttggtgataaggcaacactgcacttttctgaaaagtcttaccacagaatttacacctcttagaaaaagaatgagtcttcaataaacttgtttatctgagcaaccataacatggttaagcttttccgttcatatgatgtacatcatataaaatcaacaggcaaatgggcattctaatattttcattactgaacattctatttcagataatcataaaacaaacccaattcgtgttacctaaatggaagtgatctagatgtggaagatctttagacaaatctggaaaaaagaaatacaggcatttttttcctttataggagacccttgcgtaagtgtgacccgaagtaattccaaacagactaggtttttcattttacaaaatttgtgtattttttttatgtcacatgtcaaggcctacatcccatagccatacacatagatacaggaattcttaaaaatgggggaaaaaggcatggtaattctgttaatattacaataaacaaactcaaaattcttacaggtacataagttgacaagcttttaacatccaagttttaaatatcggctttgaggaacccaaaacttttaggttactggagctacattatatccttaaaaaactaggtctaaattcacaccaataggagaacataatttgagatggaatttcatcctttagtatttctatctactaaaaaaaaaatccacttgttaacagataaggattcattgcacaaggaatgatgctcacattgtcacccttacttaatggttcatttcatcaattgcactaattctaaattcaaacaaacaaacaaacaaacaaacattaagctgccccctatcccaccccactgcaaataagcaacagaaatctagccagaaacttcaggagtctgtgtgaaaagaagcctccagcatactttggagaaagaaatgtttttataagaccatctgtattcatccatgtcattgctcaaagatagtttaggaaaataaagagtttggggaagcaaattaagaatgaatggtcatcctaaccagatatggaataacagtctgcatacttaatatattcagttccgacatttattaaaaagtttccatatagaaagattttttaatagatgcagaaaaactgggttcccaattcagactaccctatgtgacttttgtcattatcatcttttctgattcttacaaagtaaacctaattaagaacctccctcattagtcttccagaaaaattagcacagcttatgctaattactcctgcaaaatttaataaactcgttgaaatgggaatagtctaatgaggttttatttattgaactaagataactccaaggaaaaaggttaggacacaaggatatccaatgtggtaataaaactcctatttattcaatttctaaacatgaagtttattgcaaaccttttaaattcaaatattagttactgtgtcaatatgtaaaatcaatctccaccttaattcaataactggaagtcattttttgctttttactttaacaataattaccacacatagccctttacctcaaaaataatgaaatctgctgttatcagttcctggttatttgctattaaacataacacatttgacttttcccatgtctatgcagctcaaatatctggatcactgagtgcaggctgggttatgtgcttcttaatcaagctatttggcaccacacagaaatgtaacctggcattcaactccagatgtgcacttcctgcatttacagcaatttttctataaacttttttgaagtgacttgacaaattgtcatgattgtaaaaagaattggggtcatatgtttctcagtctgtgcatgccataaggatgaagtataatagaagccccttttctaaatcacagtttgcaactgctgattttgttaattctacttttttgatagaatatgccaggctgatgtcccaaagtcagtggcagcaaataatacagccaaaatttaacacagaaatagcttgccctgcacgattgcactatgaccagaaagtctcttctctctaccctataaatagttttcctgaataaaccactgctaaaagtcttttgactgataaaaatagtagtgttctcccaaattccgaaggacaagcaaagagagctaaaaattattggtgctcaaaagttgactgcgtgttaaaactatgctaaatcctaacgcaaggatggcctgtaccctcagctctgtaattgcatattgtatgcatcttttgaaaacagttactattgctactgaatgcaggcctcatagcctattttcacaaaatattcagggatttgcatccataaatctgaaagcaaatcaaaccctaagcacgtaacacagatattatgcaatcagtaatatagaatcaaattggaaactatgaaattcaaacacggttgccatcattttttcccctttgcagcaattttatggaattgaaaaatcttttctattttgccctttcttgcataagttcttctcttgttgttattctcttctctcgctgttaagaatgggagtttcacatatcagcacagacaggactggagcttttaaaacctttggcagcctgaaggacaaataaattctgaaaactcaggtgcaaataaaaatagctaaatggggttttgcatatcaactggcatcactgcatgaaaagatagttcatcagaaacaatggcaacagccagcgaataaacatatgctgtggggcttgtgcacatacactgagtttcagctgtttttaaagtactcctatctgaagagaccaagattggctacacactgttttctactttgtcaaaccaaaagggaaaaaaaatgaaaaggataaatgtcatgagtaatatccccaaagccaccaacagcataaagtgcatacttattttgcctaaattgtttgaactaccccagccaagaaaaggttttaagtacccttctgggacagatgcaaagcggcaacaatagaagccacactaatgcaatccaggtaacacaatcctgtttcaaaaacaggggccgggctaattacagtgctgctgagtcaagtttcttatgccatcgcaacccacaggaacaggtcaaaatcaaatgttattcaaaccacagtcatatcaaccttctatatcagagtcacagcttcaaaccaaacgaagaacttaaaagcttaacccattcacaagcgaaaaaaaaaaaaaagtcttttcattgagggtggcaaggtaaggttcttgtcatcatctaaaccaaaaggaactacatggcagaacaaaatgcttatagtttcaaagttttggggactatttgggctggtcctttgatccgtacactttcttttcaacagaggaggaagaaaaatgcttaaaataacaaatgatattttggagaggtaaatttaaataaaacaaaccagcataaaggttaaatttacttgtgaccttattcatttggagacttatgttcaatcacagaaaaagcaactatatgaacagtatatctgcttttgtagataaacatgttatcctaattctataggtagcacacacatcaccatatgtcaaactttctcatcttttaactttgaatcaaatatactaatactcttatatggagcaaaaatatatatattttagtgaatactagtgaggaatatttagttaaaatatctgattgaaatgtaacctttataaagcttcttggcaatcaattgggtttatgcctgaagactcacataagtcaaaatcaacaatcgatcttttggcataaattatgttgaagcgaagtaaacatcttgttttttgttgttgtcattgttaactgaaaaatgataaaacaagcccaaaaaaggtagaaagaaagatgggtttttttttcttttgttgttgttgtcaaaaatcaatattgctgaaacccaaaaagggacttgtgttcaaccattggtttcctcaatgagggatcggtcagtcttattggcaagactctttttccagctagtacaagatgctagctcttttcctagctgacaattgacagtatctataaaccttccaggccatttaactctcaatgagtaatgctatgtaacaaatggtttatcatacatgtttccatacaatgaatttcaataattaaaatgtaaaatgaatatttggaatgcgactttgcataatgcgtgcacactgactcaaaattacaccgaacaactaaaacagatttattgttctacggtgatttacttggtcatgtcagattagtaatatggatctgtttaaaaacacaaaaattaagacaagcaggataaattaatcaacttacaatatggtctcatactgcaatcaaatccggcaaataacagtagaaaatcttggttcacagatctctttaaactgcttttatgcataaataaaaccttaaagtgtagatggattacgtccaacagaactactgtagctaaaagtgataatgattcaaacatttttcaaataaaagttaaatatttataagcacccaaccacatttcataaatcacaaactattattattttatttctgaagcttcctggcacagcatgaggattgagccacagaaagtcaggaaagaaaaaatatattcctttaggagcatgaatcagacaaaaaccggagcaatccaaggaacaggcctctaaaagaacattccatatggctttcccaggaatcaaaatcgctcagcacagcgtaagtcatgaccaacaggcaaatttcagccacatgcattcctaaccctcgcccatgagcaacacaagggcaggtgtttcattataatgaggaataagaatccagtgaaagaagagtggt

SEQ ID NO: 16319 - RNA, 1507 nt, Homo sapiens
  source 1..1507: mol_type = other RNA
gggctagggcctgctgccccctccctcccagcagtccacggggcctcagacttggggcggctgaaagtgctgagggtcaggcccctggcccaggccaggttcctaagaggaaagtcgagtgggaggctgggggcctggaaaacatgggcgtggcccatggtgtcccgaggtggggacggggcaggggtgccctgtcatgtggcccaggaaatggccgcactgtgctccttggccttcatgcggagggccgcgatgctcgaggtcttgcggtccggctcgccgttgagctcgtagccattgaggcctgggctgaggctggctgctccaaacaggctgcccatgtgcgtctggcccacgtgactgccagccccagacacactcaggaagtcggtgacgctgctggccccagagccaggggggtgggcatgaggggacatgcaggcaggcaccgggtcgcaggggaccacgcaggctggcactggtgaggcagccccgttgttgccgagccaggacgggttctgaatctgggcgtagttctcagctcgggtgaggaggggcagctcatatgcagtggagaagtgggttcgaacctgctgcatctgcccaaaacgctcccgcttcctccacttggcccttcggttctggaaccagacctgcacgcgggcctcagtgaggtctgtcctcatggccagctgttcccgcgcatacacgtctgggtagtgggtcttctggaagaccttctccagctcctccagctggtagctggtgaaggtggtccggttccgccgcttcttgcccttgttgctctctgagtcggccttctccaatgggctggggaggtctgagctggcccggtcctggggccccttcaccccagcctccttgacactcaggtagctgctgtccatccccacagtgtcagagtcagggggtaactctggctcacccagggagctctctttagcgtagcagggaacctgcaaggccgcgctgtggccgctgctgccttcctggagtttgaggctgccgtccgggggcgtcttgcaggcgcctcgctgcaagtaaagatgcggttgcgcgggcggctggggctgcggctgctgctgctgcggctgcggctgcggcggcggctggggctgcggggtcgacggctggggctggaacttgttaaaggagccccgcgccccagctccactctccaggggtgtcgccaggtcctgctgcccagcgccgtaacgggcccggctcttggcgtccccgaatccctgtgctttggcggcggccgacaggaaagttgtgccgaacttgtcgcctccgggaaatgccctaaaaggcgacgagccctcccgactctgcgacaccgggctgtagtaggcgtccatggcagcggccggcgactcgcagtaagagacgcaagtctcagcattcatgcctggcttgcgcaggcggcgggcggggacgcgagcgagggcgcgaggacgccaccgcgcgccttggctgggagttt

SEQ ID NO: 16320 - RNA, 271 nt, Homo sapiens
  source 1..271: mol_type = other RNA
ggggagcgaggggcggggcgtcggggcagggcggggagccgggggcggggccgagcaccgcggccaatctccgcccgcggcccaaagcgaaaggaagggctggcgagcgcggggccgggccgcgaccgcggaggagcagtgcgtggagccccgggcctcggagcccaggcaggggcgggaagggccgggagcgggtgtgcaggctgggtgcacaggccgcctccaccgtttcgggaaagtccgtctgattctccacgcattcttgagggct

SEQ ID NO: 16321 - RNA, 3836 nt, Homo sapiens
  source 1..3836: mol_type = other RNA
ggggaggtgtgcagggctggctcacggcaggtgacatggcagggttttcttggccagcaggaactggcactgtttctaaacacagggcaacctgtgccacaggtgccacctcagcacctccagccgtcccggccacatctgcatgttttgctagctcctgctcctggaccagctgttcctggtacttcttcatgtcatactcaagctctgatgccagctgtttgtcaactgcaaagaagtccttgagctcatctcggtaatcctgcatcacctccctgagatagtgcatgagttcccgcaaagctgggatcttatttttctccagcacagtcttcagggagatgataattggaataatattttctatgaaattcctcttctgaacttgtgagatgagcttcttctgagcttcctgcatgactacatttgccaaggccatgtcatcttcttccataaggaggtctttgtctggtttagatctcattgccaaaagcttgatctcctttgagctgaggacctcaaacgtgtctgagagtaactcactggcgtccaggtccaggggtaggatgccatcagcaaagcacgccaaaatactaaggcagattttggaagtgatgttgaatcgctgttcatctgtgaagtgctctagaagaaatttgtagattttcattcgtctctctttgtttgactttcccttcaatgaaaacagccgcttctctctctctgactgggggaacttgttgtacttctcatgcttctcatagttattaaagtgaaaaatacattcaatgaagtgttggaagaacatgacagggttcctcttcagtaacaggtgagccaggcaaaactccccgaagctggcaatgtctgggtgtgaatcgatcagagtgctgacaaatcggaagaacagggagcccttccatttcacaaattcctcctgcaagagattggtaagcaagatgagtgtctgcttccggatgaatgggtcggaatccttcagacacatggagatgttgggaatatacttgtccaccatgatggtgtagcgaatgcagagatcgcacattacaatgatgacgttgttgcggacagccacgtcctcacacacctcgagctctcgcaccagggctgggatgctcttctttgccagatcctcgtgctgtaagcacagcttacctaaggtaatgatggcatgtgctctaatcacagagggcatgacagaacctctgacctgggggggtggctgagacgctggggcctcactgctgccttgagatgatggtgagtggtcagcatcagcagacgaagccaggacggactgaatcagaaggaagatgcgcttctccaccctggctggacacagctgggctatatcccctaaggtaaaaatgtacttcaccaacaggtcttcgtccatattccctgttccattctccttgagaacgatgttggagaggcggtgctcgcaggtggagagtacatccccacacacctgcgtcagcaattcctgctcctctgctggtgtctctgcagatgctctacaaagcctctgcaaggcgtcaacagctgaactgatcacctctagagaccactgaaatccattcagcttacacttgacagcatcagtcactttgtcccgggtgctcttaggaagatgctttgcaatatgcccaatcacacagagaatatgtcctaaggtgtttgaattgggattctgctgactgctgattttctcccaagattgtattattctgctgtagtccagcctgggtgaggagccagcaatcttggagagcagcatccaggcaggtgccgaatgttccgtgccagtgtgagatattacattgtttataaaagtgggtgagaatttttctttcttggaccagatatgaaaagccttatttaaatatcggctcagttcctggctttcggtggtgaggagagtaagaagcgcccaggcgaggacctggctgtcgtccccagagtgaaaatgactgtgatgccggatgttctgcagcagcagctggtccaggaactccagggccttctcctgcacagtgctctcgcagtccatcaccaccgggaccaccccccgcaaccaggctttctggatctgcacgcatctaggctgagccataaggagttcagtaagagactggagggcctgcttccggacagacactgcagggtcccgacactggtcctgcagaatccacaggtcttccttcatgcctgagacatcacagtgtttcaaaatactcactaatacctgcagtgcagacttcctaacgttggtcttctcatccctgatcctccttctcagcattgccatgacacatctttctccagatccaactgtttcaccactgctgtctatgttgatctcccctgagggttcggaacggttagatgtctgcctttggtaggaaaaagctgatgaatttctcagtaaggtaccagggtgactctctattacagaaaacgtaggactgttaatcaggagctccaggatactctccgacgcactggtaacagtcaactccagacagtgtgcaaagctggacagtgccttgctgcggacagtaggcgccttgtctaagcaacgatcaaacataatttcctgcaccaggaacttatgctttaagaacttctgatgctccaaggagagggtgttatccacctctctttcaggcagttctaacagagctaagacaacatcaagagtaaaaacccggtgtgggatcttggaacttcgggagtatttgtaaagccaggcaatgaacatagcgtattccccacaaggaagtttactgagcagctggactagggactgggctgcaaaagtacgatactctgatttatctaccaccttggcacagatgtgctgcagtaagatacggacgactgggaatatactctcctttaattcatccacaagggcgctgataaactggaccgcctggtttctacagttgatgacttgggaggtaacagcaaggggggcacgatgggatccttcaccaacttctaacattaatattacactgagcatttgatggaaaacacaactgatgaccttatctccttctccatgaatgggagagcacagcaaatacaatccataataagccagttctggtatgtattttgcttggttaagagctctggcttgtgtaacatgacattcatgaagaactggctcaaaattagttaatgaaacaaagacctctatacaattctgtacacattgtggcttttctttcaaggaaaactttggcagaagccttaaaaaattctttaaaaggtgaaagatggcatttcgaatttgagaaaggtcccgggcagaaaaacaaatattctcatcttcttgttcttctataatttcatccatctcaatatcttctctcctgggtggctttcccctttttctatgcctcccggggttagcctgagagctcttaggctgttctttctttcttttccgattcaagttagattcctggggccagctcttctttagagtctgaatgcatttgtcaaacatcactgggtggaatacttgattggctacactgcctccatagatccatgttctccagtagcaaagggtaaaaggctttcatagagttttgtgaatgcagccaatccagtctctatgatctctgcttctatgctgggatccaaaggctcagtctctgtgaaatccagttcccacactgtgtcaacccattcgagtctaagatccagcggacaccagggctgcaggccgctaccaaggccccgcaacgccaccatgatcccagggcaccggctcgccgccgccgtgctcaactttc

SEQ ID NO: 16322 - RNA, 3999 nt, Homo sapiens
  source 1..3999: mol_type = other RNA
ggggaggtgtgcagggctggctcacggcaggtgacatggcagggttttcttggccagcaggaactggcactgtttctaaacacagggcaacctgtgccacaggtgccacctcagcacctccagccgtcccggccacatctgcatgttttgctagctcctgctcctggaccagctgttcctggtacttcttcatgtcatactcaagctctgatgccagctgtttgtcaactgcaaagaagtccttgagctcatctcggtaatcctgcatcacctccctgagatagtgcatgagttcccgcaaagctgggatcttatttttctccagcacagtcttcagggagatgataattggaataatattttctatgaaattcctcttctgaacttgtgagatgagcttcttctgagcttcctgcatgactacatttgccaaggccatgtcatcttcttccataaggaggtctttgtctggtttagatctcattgccaaaagcttgatctcctttgagctgaggacctcaaacgtgtctgagagtaactcactggcgtccaggtccaggggtaggatgccatcagcaaagcacgccaaaatactaaggcagattttggaagtgatgttgaatcgctgttcatctgtgaagtgctctagaagaaatttgtagattttcattcgtctctctttgtttgactttcccttcaatgaaaacagccgcttctctctctctgactgggggaacttgttgtacttctcatgcttctcatagttattaaagtgaaaaatacattcaatgaagtgttggaagaacatgacagggttcctcttcagtaacaggtgagccaggcaaaactccccgaagctggcaatgtctgggtgtgaatcgatcagagtgctgacaaatcggaagaacagggagcccttccatttcacaaattcctcctgcaagagattggtaagcaagatgagtgtctgcttccggatgaatgggtcggaatccttcagacacatggagatgttgggaatatacttgtccaccatgatggtgtagcgaatgcagagatcgcacattacaatgatgacgttgttgcggacagccacgtcctcacacacctcgagctctcgcaccagggctgggatgctcttctttgccagatcctcgtgctgtaagcacagcttacctaaggtaatgatggcatgtgctctaatcacagagggcatgacagaacctctgacctgggggggtggctgagacgctggggcctcactgctgccttgagatgatggtgagtggtcagcatcagcagacgaagccaggacggactgaatcagaaggaagatgcgcttctccaccctggctggacacagctgggctatatcccctaaggtaaaaatgtacttcaccaacaggtcttcgtccatattccctgttccattctccttgagaacgatgttggagaggcggtgctcgcaggtggagagtacatccccacacacctgcgtcagcaattcctgctcctctgctggtgtctctgcagatgctctacaaagcctctgcaaggcgtcaacagctgaactgatcacctctagagaccactgaaatccattcagcttacacttgacagcatcagtcactttgtcccgggtgctcttaggaagatgctttgcaatatgcccaatcacacagagaatatgtcctaaggtgtttgaattgggattctgctgactgctgattttctcccaagattgtattattctgctgtagtccagcctgggtgaggagccagcaatcttggagagcagcatccaggcaggtgccgaatgttccgtgccagtgtgagatattacattgtttataaaagtgggtgagaatttttctttcttggaccagatatgaaaagccttatttaaatatcggctcagttcctggctttcggtggtgaggagagtaagaagcgcccaggcgaggacctggctgtcgtccccagagtgaaaatgactgtgatgccggatgttctgcagcagcagctggtccaggaactccagggccttctcctgcacagtgctctcgcagtccatcaccaccgggaccaccccccgcaaccaggctttctggatctgcacgcatctaggctgagccataaggagttcagtaagagactggagggcctgcttccggacagacactgcagggtcccgacactggtcctgcagaatccacaggtcttccttcatgcctgagacatcacagtgtttcaaaatactcactaatacctgcagtgcagacttcctaacgttggtcttctcatccctgatcctccttctcagcattgccatgacacatctttctccagatccaactgtttcaccactgctgtctatgttgatctcccctgagggttcggaacggttagatgtctgcctttggtaggaaaaagctgatgaatttctcagtaaggtaccagggtgactctctattacagaaaacgtaggactgttaatcaggagctccaggatactctccgacgcactggtaacagtcaactccagacagtgtgcaaagctggacagtgccttgctgcggacagtaggcgccttgtctaagcaacgatcaaacataatttcctgcaccaggaacttatgctttaagaacttctgatgctccaaggagagggtgttatccacctctctttcaggcagttctaacagagctaagacaacatcaagagtaaaaacccggtgtgggatcttggaacttcgggagtatttgtaaagccaggcaatgaacatagcgtattccccacaaggaagtttactgagcagctggactagggactgggctgcaaaagtacgatactctgatttatctaccaccttggcacagatgtgctgcagtaagatacggacgactgggaatatactctcctttaattcatccacaagggcgctgataaactggaccgcctggtttctacagttgatgacttgggaggtaacagcaaggggggcacgatgggatccttcaccaacttctaacattaatattacactgagcatttgatggaaaacacaactgatgaccttatctccttctccatgaatgggagagcacagcaaatacaatccataataagccagttctggtatgtattttgcttggttaagagctctggcttgtgtaacatgacattcatgaagaactggctcaaaattagttaatgaaacaaagacctctatacaattctgtacacattgtggcttttctttcaaggaaaactttggcagaagccttaaaaaattctttaaaaggtgaaagatggcatttcgaatttgagaaaggtcccgggcagaaaaacaaatattctcatcttcttgttcttctataatttcatccatctcaatatcttctctcctgggtggctttcccctttttctatgcctcccggggttagcctgagagctcttaggctgttctttctttcttttccgattcaagttagattcctggggccagctcttctttagagtctgaatgcatttgtcaaacatcactgggtggaatacttgattggctacactgcctggtacttctagtagcaaaaagtaaagcccagcggcatgaaggccatattctcgatactgtacactgacattcttcttatgaactatttgaacaaaatgatagaacaatgccaccagtgtactatgggaaacattgttctcaatgaagaaggtccagatactctccatagatccatgttctccagtagcaaagggtaaaaggctttcatagagttttgtgaatgcagccaatccagtctctatgatctctgcttctatgctgggatccaaaggctcagtctctgtgaaatccagttcccacactgtgtcaacccattcgagtctaagatccagcggacaccagggctgcaggccgctaccaaggccccgcaacgccaccatgatcccagggcaccggctcgccgccgccgtgctcaactttc

SEQ ID NO: 16323 - RNA, 4498 nt, Homo sapiens
  source 1..4498: mol_type = other RNA
ggggaggtgtgcagggctggctcacggcaggtgacatggcagggttttcttggccagcaggaactggcactgtttctaaacacagggcaacctgtgccacaggtgccacctcagcacctccagccgtcccggccacatctgcatgttttgctagctcctgctcctggaccagctgttcctggtacttcttcatgtcatactcaagctctgatgccagctgtttgtcaactgcaaagaagtccttgagctcatctcggtaatcctgcatcacctccctgagatagtgcatgagttcccgcaaagctgggatcttatttttctccagcacagtcttcagggagatgataattggaataatattttctatgaaattcctcttctgaacttgtgagatgagcttcttctgagcttcctgcatgactacatttgccaaggccatgtcatcttcttccataaggaggtctttgtctggtttagatctcattgccaaaagcttgatctcctttgagctgaggacctcaaacgtgtctgagagtaactcactggcgtccaggtccaggggtaggatgccatcagcaaagcacgccaaaatactaaggcagattttggaagtgatgttgaatcgctgttcatctgtgaagtgctctagaagaaatttgtagattttcattcgtctctctttgtttgactttcccttcaatgaaaacagccgcttctctctctctgactgggggaacttgttgtacttctcatgcttctcatagttattaaagtgaaaaatacattcaatgaagtgttggaagaacatgacagggttcctcttcagtaacaggtgagccaggcaaaactccccgaagctggcaatgtctgggtgtgaatcgatcagagtgctgacaaatcggaagaacagggagcccttccatttcacaaattcctcctgcaagagattggtaagcaagatgagtgtctgcttccggatgaatgggtcggaatccttcagacacatggagatgttgggaatatacttgtccaccatgatggtgtagcgaatgcagagatcgcacattacaatgatgacgttgttgcggacagccacgtcctcacacacctcgagctctcgcaccagggctgggatgctcttctttgccagatcctcgtgctgtaagcacagcttacctaaggtaatgatggcatgtgctctaatcacagagggcatgacagaacctctgacctgggggggtggctgagacgctggggcctcactgctgccttgagatgatggtgagtggtcagcatcagcagacgaagccaggacggactgaatcagaaggaagatgcgcttctccaccctggctggacacagctgggctatatcccctaaggtaaaaatgtacttcaccaacaggtcttcgtccatattccctgttccattctccttgagaacgatgttggagaggcggtgctcgcaggtggagagtacatccccacacacctgcgtcagcaattcctgctcctctgctggtgtctctgcagatgctctacaaagcctctgcaaggcgtcaacagctgaactgatcacctctagagaccactgaaatccattcagcttacacttgacagcatcagtcactttgtcccgggtgctcttaggaagatgctttgcaatatgcccaatcacacagagaatatgtcctaaggtgtttgaattgggattctgctgactgctgattttctcccaagattgtattattctgctgtagtccagcctgggtgaggagccagcaatcttggagagcagcatccaggcaggtgccgaatgttccgtgccagtgtgagatattacattgtttataaaagtgggtgagaatttttctttcttggaccagatatgaaaagccttatttaaatatcggctcagttcctggctttcggtggtgaggagagtaagaagcgcccaggcgaggacctggctgtcgtccccagagtgaaaatgactgtgatgccggatgttctgcagcagcagctggtccaggaactccagggccttctcctgcacagtgctctcgcagtccatcaccaccgggaccaccccccgcaaccaggctttctggatctgcacgcatctaggctgagccataaggagttcagtaagagactggagggcctgcttccggacagacactgcagggtcccgacactggtcctgcagaatccacaggtcttccttcatgcctgagacatcacagtgtttcaaaatactcactaatacctgcagtgcagacttcctaacgttggtcttctcatccctgatcctccttctcagcattgccatgacacatctttctccagatccaactgtttcaccactgctgtctatgttgatctcccctgagggttcggaacggttagatgtctgcctttggtaggaaaaagctgatgaatttctcagtaaggtaccagggtgactctctattacagaaaacgtaggactgttaatcaggagctccaggatactctccgacgcactggtaacagtcaactccagacagtgtgcaaagctggacagtgccttgctgcggacagtaggcgccttgtctaagcaacgatcaaacataatttcctgcaccaggaacttatgctttaagaacttctgatgctccaaggagagggtgttatccacctctctttcaggcagttctaacagagctaagacaacatcaagagtaaaaacccggtgtgggatcttggaacttcgggagtatttgtaaagccaggcaatgaacatagcgtattccccacaaggaagtttactgagcagctggactagggactgggctgcaaaagtacgatactctgatttatctaccaccttggcacagatgtgctgcagtaagatacggacgactgggaatatactctcctttaattcatccacaagggcgctgataaactggaccgcctggtttctacagttgatgacttgggaggtaacagcaaggggggcacgatgggatccttcaccaacttctaacattaatattacactgagcatttgatggaaaacacaactgatgaccttatctccttctccatgaatgggagagcacagcaaatacaatccataataagccagttctggtatgtattttgcttggttaagagctctggcttgtgtaacatgacattcatgaagaactggctcaaaattagttaatgaaacaaagacctctatacaattctgtacacattgtggcttttctttcaaggaaaactttggcagaagccttaaaaaattctttaaaaggtgaaagatggcatttcgaatttgagaaaggtcccgggcagaaaaacaaatattctcatcttcttgttcttctataatttcatccatctcaatatcttctctcctgggtggctttcccctttttctatgcctcccggggttagcctgagagctcttaggctgttctttctttcttttccgattcaagttagattcctggggccagctcttctttagagtctgaatgcatttgtcaaacatcactgggtggaatacttgattggctacactgcctggtacttctagtagcaaaaagtaaagcccagcggcatgaaggccatattctcgatactgtacactgacattcttcttatgaactatttgaacaaaatgatagaacaatgccaccagtgtactatgggaaacattgttctcaatgaagaaggtccagatactcttgaagcttttggaggaaagctcttaggatattccaataaattaaccacattctttatgttactcatattgtactccctgtgaactgtacaccaagaaagctccatagatccatgttctccagtagcaaagggtaaaaggctttcatagagttttgtgaatgcagccaatccagtctctatgatctctgcttctatgctgggatccaaaggctcagtctctgtgaaatccagttcccacactgtgtcaacccattcgagtctaagatccagcggacaccagggctgcaggccgctaccaaggccccgcaacgccaccatgatcccagggcaccggctcgccgccgccgtgctcaactttcaaagctcgctcccgcgcgcgcgccgagtcgttccgagacccgcccggcccggcggtgcgatgagcttcttcggcttcgggcagagcgtggaggtggaaatccttctgaacgatgcagagagtaggaagcgggccgagcacaagacggaggacgggaagaaggagaaatatttcctcttctacgacggggagacggtctccgggaaggtgagccttgccctcaagaaccccaacaagcggctggagcaccagggcatcaagatcgagttcatcgggcagatcggtgagtcgacccccgggaccccctcccccagcgccgacagccggccggggagcagggtgattcagggcccagctcctccggcgaggcctgtcacagtcgcttgtcaactgcagtct

SEQ ID NO: 16324 - RNA, 1892 nt, Homo sapiens
  source 1..1892: mol_type = other RNA
ggggaggtgtgcagggctgggttagaattcatctccagcagccataccttgaagttgtcatcaatcaggaagtcacagccaatgaggtcaaagtaacccagcttgcagtccagcttgggcttggcggccagaaagcagtgggccatgatctgctgcatccgcttcttgagggtggtgaagacccagtccttggcgaggccccgggccttccagaacgtgtcactgatgtagcggttgaggtgttccatgctccacaccgtgtgctccttcagcagcatgtacagagggctcttcttctgcatgaactgggggcacacggtgcctggttggtcaagtggccgccgaggtcgctggaatgggggtcgtaaaggctaagggtgaggcgagcatagccgtggccaaagaagatcatgtagggtgtggtgcaggcaatgagcaggtaggagcgcacgtcaaactttctcccgtccaccagcagcgggttctggatgtacctctgcaccacccgcgcctgaggcccccggaacggcgtcttgtggtggatggggtcgtcctccatgctccgggtcttggcctgcagggcggcaacttcctcctggttccggagcaggaagatgcctttgccctggttggaggctgtgggcttgcagatccatatctgggtttcatcaaacaaggtgaaaaaggcctctctctcgtgtttgaggtccaggcggtaggtctctgggaaaaactcttccattctcaggaccctctgtggcctgaggtatcctgggcttgtccacgggaggtcctccagggcgggcgctgctgcgtccttttccagcctggcctggaccccccccggcaccttgctggccttgctcatggcccgtgcccgtccccgaagggtgctgagcagcccgatcttggtggtgaggagcttgttgttgggaagctggtacagcagctgctctccttcccggaagctgccgtagctgtctcggctcttgacctcacaccacttcagcgtgtagtcgtcccggcggctgtcatggatgcgctgccagcccttgcttttgcagtaggagctgatgattgtggccccgttgctgcctccaatgtagaagaagggccccggccgggtgctgtggggcgatggcttcccaccccccagcaggagcccctccaggagggcagctgagggcccggcggcgttagtgtcatccgagtctgcaggccggtggctgttcaggagcccagggggtccgggtgtggcagaggctctttctgccccctccaggtccggcccacagtgtccatctgcgtcgtggtctggctggcttggctgacaccggagtccctcctcctggctgctccccattggcctctcgtgggccgggccaacagggcagtggcctggtgcagggcaggggccgggctgtgaggccggtgctgggtgcagacgtgacgcagggatggtccctgagactcgagcccgaggcctctgctggatccttggcctcttgcccctcttgaagccggctcgggtccgagtgggtggtccccggcggtggatgaaccgggtgcagctgtggtccattggccggggggtgcccgggcgagggccctgaagggaagatgccgctctgaccctcctgtgggacctccgcgcggcccgaggccccagtgcttggatggagcaggcagtcaggcccaccctgcccaggaaagggcgcctcccagggccgtgggcttgagcctctgcgtgcggctggctcccgtctctgtggcagctgtggggcctggcgccgtgtgggggcgaggctgtctctgcaccctgtctctgccgggcatgtcctccctggccggagcggctcttcaggtgtggctgagctcggcctgggtgccgg

SEQ ID NO: 16325 - RNA, 1550 nt, Homo sapiens
  source 1..1550: mol_type = other RNA
ggggaggtgtgcagggctgggttagaattcatctccagcagccataccttgaagttgtcatcaatcaggaagtcacagccaatgaggtcaaagtaacccagcttgcagtccagcttgggcttggcggccagaaagcagtgggccatgatctgctgcatccgcttcttgagggtggtgaagacccagtccttggcgaggccccgggccttccagaacgtgtcactgatgtagcggttgaggtgttccatgctccacaccgtgtgctccttcagcagcatgtacagagggctcttcttctgcatgaactggttggtcaagtggccgccgaggtcgctggaatgggggtcgtaaaggctaagggtgaggcgagcatagccgtggccaaagaagatcatgtagggtgtggtgcaggcaatgagcaggtaggagcgcacgtcaaactttctcccgtccaccagcagcgggttctggatgtacctctgcaccacccgcgcctgaggcccccggaacggcgtcttgtggtggatggggtcgtcctccatgctccgggtcttggcctgcagggcggcaacttcctcctggttccggagcaggaagatgcctttgccctggttggaggctgtgggcttgcagatccatatctgggtttcatcaaacaaggtgaaaaaggcctctctctcgtgtttgaggtccaggcggtaggtctctgggaaaaactcttccattctcaggaccctctgtggcctgaggtatcctgggcttgtccacgggaggtcctccagggcgggcgctgctgcgtccttttccagcctggcctggaccccccccggcaccttgctggccttgctcatggcccgtgcccgtccccgaagggtgctgagcagcccgatcttggtggtgaggagcttgttgttgggaagctggtacagcagctgctctccttcccggaagctgccgtagctgtctcggctcttgacctcacaccacttcagcgtgtagtcgtcccggcggctgtcatggatgcgctgccagcccttgcttttgcagtaggagctgatgattgtggccccgttgctgcctccaatgtagaagaagggccccggccgggtgctgtggggcgatggcttcccaccccccagcaggagcccctccaggagggcagctgagggcccggcggcgttagtgtcatccgagtctgcaggccggtggctgttcaggagcccagggggtccgggtgtggcagaggctctttctgccccctccaggtccggcccacagtgtccatctgcgtcgtggtctggctggcttggctgacaccggagtccctcctcctggctgctccccattggcctctcgtgggccgggcatctggggaggggccgtgaccaccctccagggccaggcttcctgccggcaggttccaggtgggggtggggagcttggagcagggggcagggaggtcgcccctccgaccctcctcaccaacagggcagtggcctggtgcagggcaggggccgggctgtgaggccggtgctgggtgcagacgtgac

SEQ ID NO: 16326 - RNA, 1647 nt, Homo sapiens
  source 1..1647: mol_type = other RNA
ggggaggtgtgcagggctgggttagaattcatctccagcagccataccttgaagttgtcatcaatcaggaagtcacagccaatgaggtcaaagtaacccagcttgcagtccagcttgggcttggcggccagaaagcagtgggccatgatctgctgcatccgcttcttgagggtggtgaagacccagtccttggcgaggccccgggccttccagaacgtgtcactgatgtagcggttgaggtgttccatgctccacaccgtgtgctccttcagcagcatgtacagagggctcttcttctgcatgaactggttggtcaagtggccgccgaggtcgctggaatgggggtcgtaaaggctaagggtgaggcgagcatagccgtggccaaagaagatcatgtagggtgtggtgcaggcaatgagcaggtaggagcgcacgtcaaactttctcccgtccaccagcagcgggttctggatgtacctctgcaccacccgcgcctgaggcccccggaacggcgtcttgtggtggatggggtcgtcctccatgctccgggtcttggcctgcagggcggcaacttcctcctggttccggagcaggaagatgcctttgccctggttggaggctgtgggcttgcagatccatatctgggtttcatcaaacaaggtgaaaaaggcctctctctcgtgtttgaggtccaggcggtaggtctctgggaaaaactcttccattctcaggaccctctgtggcctgaggtatcctgggcttgtccacgggaggtcctccagggcgggcgctgctgcgtccttttccagcctggcctggaccccccccggcaccttgctggccttgctcatggcccgtgcccgtccccgaagggtgctgagcagcccgatcttggtggtgaggagcttgttgttgggaagctggtacagcagctgctctccttcccggaagctgccgtagctgtctcggctcttgacctcacaccacttcagcgtgtagtcgtcccggcggctgtcatggatgcgctgccagcccttgcttttgcagtaggagctgatgattgtggccccgttgctgcctccaatgtagaagaagggccccggccgggtgctgtggggcgatggcttcccaccccccagcaggagcccctccaggagggcagctgagggcccggcggcgttagtgtcatccgagtctgcaggccggtggctgttcaggagcccagggggtccgggtgtggcagaggctctttctgccccctccaggtccggcccacagtgtccatctgcgtcgtggtctggctggcttggctgacaccggagtccctcctcctggctgctccccattggcctctcgtgggccgggccaacagggcagtggcctggtgcagggcaggggccgggctgtgaggccggtgctgggtgcagacgtgacgcagggatggtccctgagactcgagcccgaggcctctgctggatccttggcctcttgcccctcttgaagccggctcgggtccgagtgggtggtccccggcggtggatgaaccgggtgcagctgtggtccattggccggggggtgcccgggcgagggccctgatgactgtgtgccccagcctctccagctgtacagcgtcagcctctctccagc

SEQ ID NO: 16327 - RNA, 1742 nt, Homo sapiens
  source 1..1742: mol_type = other RNA
ggggaggtgtgcagggctgggttagaattcatctccagcagccataccttgaagttgtcatcaatcaggaagtcacagccaatgaggtcaaagtaacccagcttgcagtccagcttgggcttggcggccagaaagcagtgggccatgatctgctgcatccgcttcttgagggtggtgaagacccagtccttggcgaggccccgggccttccagaacgtgtcactgatgtagcggttgaggtgttccatgctccacaccgtgtgctccttcagcagcatgtacagagggctcttcttctgcatgaactggttggtcaagtggccgccgaggtcgctggaatgggggtcgtaaaggctaagggtgaggcgagcatagccgtggccaaagaagatcatgtagggtgtggtgcaggcaatgagcaggtaggagcgcacgtcaaactttctcccgtccaccagcagcgggttctggatgtacctctgcaccacccgcgcctgaggcccccggaacggcgtcttgtggtggatggggtcgtcctccatgctccgggtcttggcctgcagggcggcaacttcctcctggttccggagcaggaagatgcctttgccctggttggaggctgtgggcttgcagatccatatctgggtttcatcaaacaaggtgaaaaaggcctctctctcgtgtttgaggtccaggcggtaggtctctgggaaaaactcttccattctcaggaccctctgtggcctgaggtatcctgggcttgtccacgggaggtcctccagggcgggcgctgctgcgtccttttccagcctggcctggaccccccccggcaccttgctggccttgctcatggcccgtgcccgtccccgaagggtgctgagcagcccgatcttggtggtgaggagcttgttgttgggaagctggtacagcagctgctctccttcccggaagctgccgtagctgtctcggctcttgacctcacaccacttcagcgtgtagtcgtcccggcggctgtcatggatgcgctgccagcccttgcttttgcagtaggagctgatgattgtggccccgttgctgcctccaatgtagaagaagggccccggccgggtgctgtggggcgatggcttcccaccccccagcaggagcccctccaggagggcagctgagggcccggcggcgttagtgtcatccgagtctgcaggccggtggctgttcaggagcccagggggtccgggtgtggcagaggctctttctgccccctccaggtccggcccacagtgtccatctgcgtcgtggtctggctggcttggctgacaccggagtccctcctcctggctgctccccattggcctctcgtgggccgggccaacagggcagtggcctggtgcagggcaggggccgggctgtgaggccggtgctgggtgcagacgtgacgcagggatggtccctgagactcgagcccgaggcctctgctggatccttggcctcttgcccctcttgaagccggctcgggtccgagtgggtggtccccggcggtggatgaaccgggtgcagctgtggtccattggccggggggtgcccgggcgagggccctggtgagatgaaaagaccggcaggagacggcaccccggtaggatgaacagaagagacttttaaacattgttcgaagagctggtgcctcccggccggaggccgctgcccagcccacaaggtcctgggagcctgggccaggaaacaacagt

SEQ ID NO: 16328 - RNA, 1761 nt, Homo sapiens
  source 1..1761: mol_type = other RNA
ggggaggtgtgcagggctgggttagaattcatctccagcagccataccttgaagttgtcatcaatcaggaagtcacagccaatgaggtcaaagtaacccagcttgcagtccagcttgggcttggcggccagaaagcagtgggccatgatctgctgcatccgcttcttgagggtggtgaagacccagtccttggcgaggccccgggccttccagaacgtgtcactgatgtagcggttgaggtgttccatgctccacaccgtgtgctccttcagcagcatgtacagagggctcttcttctgcatgaactggttggtcaagtggccgccgaggtcgctggaatgggggtcgtaaaggctaagggtgaggcgagcatagccgtggccaaagaagatcatgtagggtgtggtgcaggcaatgagcaggtaggagcgcacgtcaaactttctcccgtccaccagcagcgggttctggatgtacctctgcaccacccgcgcctgaggcccccggaacggcgtcttgtggtggatggggtcgtcctccatgctccgggtcttggcctgcagggcggcaacttcctcctggttccggagcaggaagatgcctttgccctggttggaggctgtgggcttgcagatccatatctgggtttcatcaaacaaggtgaaaaaggcctctctctcgtgtttgaggtccaggcggtaggtctctgggaaaaactcttccattctcaggaccctctgtggcctgaggtatcctgggcttgtccacgggaggtcctccagggcgggcgctgctgcgtccttttccagcctggcctggaccccccccggcaccttgctggccttgctcatggcccgtgcccgtccccgaagggtgctgagcagcccgatcttggtggtgaggagcttgttgttgggaagctggtacagcagctgctctccttcccggaagctgccgtagctgtctcggctcttgacctcacaccacttcagcgtgtagtcgtcccggcggctgtcatggatgcgctgccagcccttgcttttgcagtaggagctgatgattgtggccccgttgctgcctccaatgtagaagaagggccccggccgggtgctgtggggcgatggcttcccaccccccagcaggagcccctccaggagggcagctgagggcccggcggcgttagtgtcatccgagtctgcaggccggtggctgttcaggagcccagggggtccgggtgtggcagaggctctttctgccccctccaggtccggcccacagtgtccatctgcgtcgtggtctggctggcttggctgacaccggagtccctcctcctggctgctccccattggcctctcgtgggccgggccaacagggcagtggcctggtgcagggcaggggccgggctgtgaggccggtgctgggtgcagacgtgacgcagggatggtccctgagactcgagcccgaggcctctgctggatccttggcctcttgcccctcttgaagccggctcgggtccgagtgggtggtccccggcggtggatgaaccgggtgcagctgtggtccattggccggggggtgcccgggcgagggccctggtgagatgaaaagaccggcaggagacggcaccccggtaggatgaacagaagagacttttaaacattgttcgaagagctggtgcctcccggccggaggccgctgtcaaaggacgcacgacctgcccagcccacaaggtcctgggagcctgggccaggaaacaacagt

SEQ ID NO: 16329 - RNA, 1793 nt, Homo sapiens
  source 1..1793: mol_type = other RNA
ggggaggtgtgcagggctgggttagaattcatctccagcagccataccttgaagttgtcatcaatcaggaagtcacagccaatgaggtcaaagtaacccagcttgcagtccagcttgggcttggcggccagaaagcagtgggccatgatctgctgcatccgcttcttgagggtggtgaagacccagtccttggcgaggccccgggccttccagaacgtgtcactgatgtagcggttgaggtgttccatgctccacaccgtgtgctccttcagcagcatgtacagagggctcttcttctgcatgaactggttggtcaagtggccgccgaggtcgctggaatgggggtcgtaaaggctaagggtgaggcgagcatagccgtggccaaagaagatcatgtagggtgtggtgcaggcaatgagcaggtaggagcgcacgtcaaactttctcccgtccaccagcagcgggttctggatgtacctctgcaccacccgcgcctgaggcccccggaacggcgtcttgtggtggatggggtcgtcctccatgctccgggtcttggcctgcagggcggcaacttcctcctggttccggagcaggaagatgcctttgccctggttggaggctgtgggcttgcagatccatatctgggtttcatcaaacaaggtgaaaaaggcctctctctcgtgtttgaggtccaggcggtaggtctctgggaaaaactcttccattctcaggaccctctgtggcctgaggtatcctgggcttgtccacgggaggtcctccagggcgggcgctgctgcgtccttttccagcctggcctggaccccccccggcaccttgctggccttgctcatggcccgtgcccgtccccgaagggtgctgagcagcccgatcttggtggtgaggagcttgttgttgggaagctggtacagcagctgctctccttcccggaagctgccgtagctgtctcggctcttgacctcacaccacttcagcgtgtagtcgtcccggcggctgtcatggatgcgctgccagcccttgcttttgcagtaggagctgatgattgtggccccgttgctgcctccaatgtagaagaagggccccggccgggtgctgtggggcgatggcttcccaccccccagcaggagcccctccaggagggcagctgagggcccggcggcgttagtgtcatccgagtctgcaggccggtggctgttcaggagcccagggggtccgggtgtggcagaggctctttctgccccctccaggtccggcccacagtgtccatctgcgtcgtggtctggctggcttggctgacaccggagtccctcctcctggctgctccccattggcctctcgtgggccgggccaacagggcagtggcctggtgcagggcaggggccgggctgtgaggccggtgctgggtgcagacgtgacgcagggatggtccctgagactcgagcccgaggcctctgctggatccttggcctcttgcccctcttgaagccggctcgggtccgagtgggtggtccccggcggtggatgaaccgggtgcagctgtggtccattggccggggggtgcccgggcgagggccctggtgagatgaaaagaccggcaggagacggcaccccggtaggatgaacagaagagacttttaaacattgttcgaagagctggtgcctcccggccggaggccgctgtcaaaggacgcacgacctgtgggctcaagcagccgtccgtccaggacttgctctgcggaggcagacctgcccagcccacaaggtcctgggagcct

SEQ ID NO: 16330 - RNA, 1794 nt, Homo sapiens
  source 1..1794: mol_type = other RNA
ggggaggtgtgcagggctgggttagaattcatctccagcagccataccttgaagttgtcatcaatcaggaagtcacagccaatgaggtcaaagtaacccagcttgcagtccagcttgggcttggcggccagaaagcagtgggccatgatctgctgcatccgcttcttgagggtggtgaagacccagtccttggcgaggccccgggccttccagaacgtgtcactgatgtagcggttgaggtgttccatgctccacaccgtgtgctccttcagcagcatgtacagagggctcttcttctgcatgaactggttggtcaagtggccgccgaggtcgctggaatgggggtcgtaaaggctaagggtgaggcgagcatagccgtggccaaagaagatcatgtagggtgtggtgcaggcaatgagcaggtaggagcgcacgtcaaactttctcccgtccaccagcagcgggttctggatgtacctctgcaccacccgcgcctgaggcccccggaacggcgtcttgtggtggatggggtcgtcctccatgctccgggtcttggcctgcagggcggcaacttcctcctggttccggagcaggaagatgcctttgccctggttggaggctgtgggcttgcagatccatatctgggtttcatcaaacaaggtgaaaaaggcctctctctcgtgtttgaggtccaggcggtaggtctctgggaaaaactcttccattctcaggaccctctgtggcctgaggtatcctgggcttgtccacgggaggtcctccagggcgggcgctgctgcgtccttttccagcctggcctggaccccccccggcaccttgctggccttgctcatggcccgtgcccgtccccgaagggtgctgagcagcccgatcttggtggtgaggagcttgttgttgggaagctggtacagcagctgctctccttcccggaagctgccgtagctgtctcggctcttgacctcacaccacttcagcgtgtagtcgtcccggcggctgtcatggatgcgctgccagcccttgcttttgcagtaggagctgatgattgtggccccgttgctgcctccaatgtagaagaagggccccggccgggtgctgtggggcgatggcttcccaccccccagcaggagcccctccaggagggcagctgagggcccggcggcgttagtgtcatccgagtctgcaggccggtggctgttcaggagcccagggggtccgggtgtggcagaggctctttctgccccctccaggtccggcccacagtgtccatctgcgtcgtggtctggctggcttggctgacaccggagtccctcctcctggctgctccccattggcctctcgtgggccgggcctgagactcgagcccgaggcctctgctggatccttggcctcttgcccctcttgaagccggctcgggtccgagtgggtggtccccggcggtggatgaaccgggtgcagctgtggtccattggccggggggtgcccgggcgagggccctgaagggaagatgccgctctgaccctcctgtgggacctccgcgcggcccgaggccccagtgcttggatggagcaggcagtcaggcccaccctgcccaggaaagggcgcctcccagggccgtgggcttgagcctctgcgtgcggctggctcccgtctctgtggcagctgtggggcctggcgccgtgtgggggcgaggctgtctctgcaccctgtctctgccgggcatgtcctccctggccggagcggctcttcaggtgtggctgagctcggcctgggtgccgg

SEQ ID NO: 16331 - RNA, 63 nt, Homo sapiens
  source 1..63: mol_type = other RNA
ggggcgcggccggatcgcggctcccctctccggtgtagtgcagaaagcttcctacttgcgacc

SEQ ID NO: 16332 - RNA, 127 nt, Homo sapiens
  source 1..127: mol_type = other RNA
ggggctggggccggggccgagcccgcggcggggccgcctcccgtccggcgggctcaggctccgcgccaggcccgggcgccgcgctctcggcctgccgtcccccctggagttggccgcgccctctctc

SEQ ID NO: 16333 - RNA, 766 nt, Homo sapiens
  source 1..766: mol_type = other RNA
ggggctggggccggggccgagcccgcggcggggccgcctcccgtccggcgggctcaggctccgcgccaggcccgggcgccgcgctctcggcctgccgtcccccctggagttggccgcgccctctctcgtccccaacgcctccgcaagtccccgccccgtttcctgccgccgcgccccgccccggcctgtccccggagcggcccggtggcgcgggcggccagagcccaggcctggaagcccggccggccccgccccgacccgggcccgcccccttggagcgcctggacgctcagcgccccctgcccgccgccgagagcgggagttggggacggacgcgcgagttggggacggagagcgggagttgcgaccggacgcgcgaggcagggccgaggccgtgtgttcagaccacgtgggcgcggggtgcgcgacagggtctgtgtcctgcgctgcgtgagccgcggtgggtgtccgcgaaacgctgtgtgtggagtgcgtgcgtgtgtccgccctcgccaggctgttggtctacaccgcccaacttactcagtcatccattcattcaacagtcttgttaactgagtgccaattacgctccaggcgctgcgaatacgagtgggtctccaccaccagaatggctaaagtgaaaaagaccgcaccgtgtggaggcgagaaagtagagcgactggacctctcttgtatttctgggggagtgtaaattggtagagacattttggaaaactggcagttttctaatgaagccgaacat

SEQ ID NO: 16334 - RNA, 957 nt, Homo sapiens
  source 1..957: mol_type = other RNA
ggggctggggccggggccgagcgcgccgcggcggggttttgctagcctttgctgtgtcctggcctcaacggcgccgcgccgggaagtttgcagggcaggcggcgggaagttatttaagcactggctcgaagtgaggacagagaactgggcagggggttacccaggccaattcttgggccattccgccccaaggaacatggagctgtccccaagctttcttgagccccgccgggcggacgcttctcggctaatctttctgcaacttttacaaagctgcctcctccccagtttgatctctgcaaacacatcctgggcgtccgcggcagcttggaaactatttttaccgtctggggccgaggagttgcattgaaataaggaaggcgaggcgccttctctagcgtttcaccccggaccaggctgggtcacccagtggcctctttgctcccccgccccacccttcgtgcgccttccagagccgccatcgaatctctcttgctaacttgcagcgctctgggggttctccagacacaggcgcaggagggagccttcgtcgaggaaagttccggctacctctgttggggaatttgctttcatttttcaccgcgggcgaacctggccaggcgggtttccgaagcactggcagaggtgggggctgccaggcactgccaggcagcgagaggccgctcgacctgggggcgccgcttgtccagcctccctcggagggcagacttgcagccacccgggcactagaaaccacctcgagtcctgcgttgggccgaggtgtcggcgtacacgcgagccgggagccgtttcttgcaggatgcctgcgagctggatgtattcggataaatgcagcgcaaacgacagccagagaaatcccgtcgattcaagggcagttccagacccgacccccgcgcgcacccggctcagccccaggtgcgcgccggtcgaaaccgg

SEQ ID NO: 16335 - RNA, 1189 nt, Homo sapiens
  source 1..1189: mol_type = other RNA
ggggctggggccggggccgagcgcgccgcggcggggttttgctagcctttgctgtgtcctggcctcaacggcgccgcgccgggaagtttgcagggcaggcggcgggaagttatttaagcactggctcgaagtgaggacagagaactgggcagggggttacccaggccaattcttgggccattccgccccaaggaacatggagctgtccccaagctttcttgagccccgccgggcggacgcttctcggctaatctttctgcaacttttacaaagctgcctcctccccagtttgatctctgcaaacacatcctgggcgtccgcggcagcttggaaactatttttaccgtctggggccgaggagttgcattgaaataaggaaggcgaggcgccttctctagcgtttcaccccggaccaggctgggtcacccagtggcctctttgctcccccgccccacccttcgtgcgccttccagagccgccatcgaatctctcttgctaacttgcagcgctctgggggttctccagacacaggcgcaggagggagccttcgtcgaggaaagttccggctacctctgttggggaatttgctttcatttttcaccgcgggcgaacctggccaggcgggtttccgaagcactggcagaggtgggggctgccaggcactgccaggcagcgagaggccgctcgacctgggggcgccgcttgtccagcctccctcggagggcagacttgcagccacccgggcactagaaaccacctcgagtcctgcgttgggccgaggtgtcggcgtacacgcgagccgggagccgtttcttgcaggatgcctgcgagctggatgtattcggataaatgcagcgcaaacgacagccagagaaatcccgtcgattcccggaaagttctcggtacccgtgcggagtgggagacagagaaagaagccggggaggggagtcaggtgggggaggggagtgagatgggccaagaggagagggcgagcataccaagggcagttccagacccgacccccgcgcgcacccggctcagccccaggtgcgcgccggtcgaaaccgggtctccaggctcggcccccgccccccacgcgggcacagactggctcccgactcccagagctcccagccccaccatttatcaaaaggacttgacaacaaaagaagagccggggcggaaaagc

SEQ ID NO: 16336 - RNA, 1185 nt, Homo sapiens
  source 1..1185: mol_type = other RNA
ggggctggggccggggccgagcgcgccgcggcggggttttgctagcctttgctgtgtcctggcctcaacggcgccgcgccgggaagtttgcagggcaggcggcgggaagttatttaagcactggctcgaagtgaggacagagaactgggcagggggttacccaggccaattcttgggccattccgccccaaggaacatggagctgtccccaagctttcttgagccccgccgggcggacgcttctcggctaatctttctgcaacttttacaaagctgcctcctccccagtttgatctctgcaaacacatcctgggcgtccgcggcagcttggaaactatttttaccgtctggggccgaggagttgcattgaaataaggaaggcgaggcgccttctctagcgtttcaccccggaccaggctgggtcacccagtggcctctttgctcccccgccccacccttcgtgcgccttccagagccgccatcgaatctctcttgctaacttgcagcgctctgggggttctccagacacaggcgcaggagggagccttcgtcgaggaaagttccggctacctctgttggggaatttgctttcatttttcaccgcgggcgaacctggccaggcgggtttccgaagcactggcagaggtgggggctgccaggcactgccaggcagcgagaggccgctcgacctgggggcgccgcttgtccagcctccctcggagggcagacttgcagccacccgggcactagaaaccacctcgagtcctgcgttgggccgaggtgtcggcgtacacgcgagccgggagccgtttcttgcaggatgcctgcgagctggatgtattcggataaatgcagcgcaaacgacagccagagaaatcccgtcgattcctggctccccagcctgcggggatggcggcaggtgggagaaggtcggggagggggcatgagtgagcctgagatgtttcttcccccatacacccatggccaggcctcttcttcgcagcctcttagccctgcttacgacccgagggggtcaaagaattgaggcgaggtttgccccaccattgacctccaggactagaagttccttggtggtgtggctcttagaagtctccgagtttggggttagggaactacagagggtggcagcctgacctccgcacgcaacacgccccgcgaggactc

SEQ ID NO: 16337 - RNA, 1621 nt, Homo sapiens
  source 1..1621: mol_type = other RNA
ggggctggggccggggccgagcgcgccgcggcggggttttgctagcctttgctgtgtcctggcctcaacggcgccgcgccgggaagtttgcagggcaggcggcgggaagttatttaagcactggctcgaagtgaggacagagaactgggcagggggttacccaggccaattcttgggccattccgccccaaggaacatggagctgtccccaagctttcttgagccccgccgggcggacgcttctcggctaatctttctgcaacttttacaaagctgcctcctccccagtttgatctctgcaaacacatcctgggcgtccgcggcagcttggaaactatttttaccgtctggggccgaggagttgcattgaaataaggaaggcgaggcgccttctctagcgtttcaccccggaccaggctgggtcacccagtggcctctttgctcccccgccccacccttcgtgcgccttccagagccgccatcgaatctctcttgctaacttgcagcgctctgggggttctccagacacaggcgcaggagggagccttcgtcgaggaaagttccggctacctctgttggggaatttgctttcatttttcaccgcgggcgaacctggccaggcgggtttccgaagcactggcagaggtgggggctgccaggcactgccaggcagcgagaggccgctcgacctgggggcgccgcttgtccagcctccctcggagggcagacttgcagccacccgggcactagaaaccacctcgagtcctgcgttgggccgaggtgtcggcgtacacgcgagccgggagccgtttcttgcaggatgcctgcgagctggatgtattcggataaatgcagcgcaaacgacagccagagaaatcccgtcgattcctggtggctgcgctgcgccgcgcgggatctcgattactgcgaaggaaaaaacactgggtgtgcaggttcccttcgcccctggagttgacagtccggccggtgtccacactcccaccggtgctccttctggacaccccccgcagtctgttcctcacgcgcaccccccttcaaaagaaggtttcagtttattttcgagctggggaaaggaagaacgacgaggaggaaaaaagagggaggcggcggatggcaaacgtagaataaatgtccatctcgtcctcccagcgaaatcgagggaggggacacacaggggggcggcgaagagggagctgcccattaaaaccggcactgagagtcctggcagcggcggcggcggcggcgcgggacgcgtcacatccccttgaccctccaatcacctcgggctcccatttgattggaaggcggcaaaggctttaatctcccccttggtgcagctgcttttgaagtgagtttcctcgccagagccccggctggacacgcagcggctcgcatcgcagagcgcagcgccggcgcggggccgcgagaacgcagcgcaggggagcagcccgaggcggacaccgcgagccgcccggcactcccgcagtccagccggctcctctagcccggccacggctccgctgcgggccacccaggattactcgcgtctggctccaggcgccgagaaggcgcgctgggcgcccgtggccgccgcgccagc

SEQ ID NO: 16338 - RNA, 1007 nt, Homo sapiens
  source 1..1007: mol_type = other RNA
ggggctggggccggggccgagcgcgccgcggcggggttttgctagcctttgctgtgtcctggcctcaacggcgccgcgccgggaagtttgcagggcaggcggcgggaagttatttaagcactggctcgaagtgaggacagagaactgggcagggggttacccaggccaattcttgggccattccgccccaaggaacatggagctgtccccaagctttcttgagccccgccgggcggacgcttctcggctaatctttctgcaacttttacaaagctgcctcctccccagtttgatctctgcaaacacatcctgggcgtccgcggcagcttggaaactatttttaccgtctggggccgaggagttgcattgaaataaggaaggcgaggcgccttctctagcgtttcaccccggaccaggctgggtcacccagtggcctctttgctcccccgccccacccttcgtgcgccttccagagccgccatcgaatctctcttgctaacttgcagcgctctgggggttctccagacacaggcgcaggagggagccttcgtcgaggaaagttccggctacctctgttggggaatttgctttcatttttcaccgcgggcgaacctggccaggcgggtttccgaagcactggcagaggtgggggctgccaggcactgccaggcagcgagaggccgctcgacctgggggcgccgcttgtccagcctccctcggagggcagacttgcagccacccgggcactagaaaccacctcgagtcctgcgttgggccgaggtgtcggcgtacacgcgagccgggagccgtttcttgcaggatgcctgcgagctggatgtattcggataaatgcagcgcaaacgacagccagagaaatcccgtcgattctccctcagatgtcgcacggacactacaaacccccttgaatgcaggtgtgctcttacacgctcacactgacaaacaccagccccaagcacacaccgcctcactcccctcttctctccaaa

SEQ ID NO: 16339 - RNA, 1074 nt, Homo sapiens
  source 1..1074: mol_type = other RNA
ggggctggggccggggccgagcgcgccgcggcggggttttgctagcctttgctgtgtcctggcctcaacggcgccgcgccgggaagtttgcagggcaggcggcgggaagttatttaagcactggctcgaagtgaggacagagaactgggcagggggttacccaggccaattcttgggccattccgccccaaggaacatggagctgtccccaagctttcttgagccccgccgggcggacgcttctcggctaatctttctgcaacttttacaaagctgcctcctccccagtttgatctctgcaaacacatcctgggcgtccgcggcagcttggaaactatttttaccgtctggggccgaggagttgcattgaaataaggaaggcgaggcgccttctctagcgtttcaccccggaccaggctgggtcacccagtggcctctttgctcccccgccccacccttcgtgcgccttccagagccgccatcgaatctctcttgctaacttgcagcgctctgggggttctccagacacaggcgcaggagggagccttcgtcgaggaaagttccggctacctctgttggggaatttgctttcatttttcaccgcgggcgaacctggccaggcgggtttccgaagcactggcagaggtgggggctgccaggcactgccaggcagcgagaggccgctcgacctgggggcgccgcttgtccagcctccctcggagggcagacttgcagccacccgggcactagaaaccacctcgagtcctgcgttgggccgaggtgtcggcgtacacgcgagccgggagccgtttcttgcaggatgcctgcgagctggatgtattcggataaatgcagcgcaaacgacagccagagaaatcccgtcgattctccgcacgcaacacgccccgcgaggactcgcggcggcggggtggggtggcgggaaatctcccgtgttagaagttgccgccgctggtctcgggtacccggagccgcgcccgaactccgcgaccccaacagaccgaggctcccagaggtggaagggcgtctctccgacaccgagagggcaggcgcaca

SEQ ID NO: 16340 - RNA, 177 nt, Homo sapiens
  source 1..177: mol_type = other RNA
gggggaagaaaaggtggggtgggggacgagctagaacggagagacaggggaaagatgagaggaggagggaaaggatcgggagggagaggaagagggtcggagagggaaggaagggagaaaaacagaggggggagagggaggcagggatagaggaggcagcgagctgcgaggagaaat

SEQ ID NO: 16341 - RNA, 7873 nt, Homo sapiens
  source 1..7873: mol_type = other RNA
ggggggtgtggagccagggggcaggtcttcagtcacagccacacggtagtgtgacaatgtgaagctcggggcgtggtcgttctggtcctgcagctgcacgtgcactgtggctcgtgctgcccggcctggagccccgtggtctcgtgcttccagcaccacatccactgctcctgacccgtcatggcccaaggccactgttcccactattgtgaacagggtcccattgttggggtcaacactgaagccatcggcaggggaagccaggtggtaggaaatgtgaccgttggcacctgagtcccgatcagtggcagagacggagagaatggcactgcctgggggtgtgtgctcaagcagcattacctggtagaggctctgtgagaaggcaggtgcattgtcattgacatcctccacaagcactgtgaggttggcacggccctcatgaggcccatcatgtgccagcagctgcagctggtagcggtcacactgctcaaagtccaggggccccgtgagggagacacggcctccatagcggccaacactgaagggatcctggggcccagatgggcttagcacataccacagcacgggtcctgagtccacatcattccctgttacctgtgcaatctctgagcccaataacgcatcttctgacactcggagctcccagggttgggggatggtggggcgattgtcattggtgtcgatgaccatcaccgtcaaggtagctgagcccaccagggctgggctccctctgtctgtggccatcagcaccaaccgtgtttcagcccagatctcacggtccaggatggctgtggtagtgatagtgcctgtggttgggtctacgtggaacaatccacgtgccggctgggatgcagccagactgtaggaaatctgtcctccagagccttgatccaggtcatccgcctccacctgcagcaggggcccctccaagggccgggactcaggaaggaaggccacataatggggccgcaggaaacggggagcattgtcgttggcatcttgcagggtcagggtcagcacagtgaaggcaaaggctcctccactctctgcctgcagcaccagtcgcagccgtggactcacctcgaagtctagcccctctgctgagcgaactgtgatggcacctgtactaggctggatggagaatgtccctttctcattcccactgagaatgctgtaggtgatgggtccatttgtgcctcctgcatggacggccctgggggagacaataggagtccctgggggcgcattctcacgaatcgtagcctcactgctagcccggggaaagcggggtccacgctcagcttccccctgcagtccaacaatgatcacaccagtggcagagcgagctggacggccaagatcagtggccacaatgaagaggacacgatctcgggggcctagagctacaggagagcgggccacgcggatttcaccagtgtaagagtccacagtagtgccaggaggtggtgtgcctgccagccggtacagaatggaagcattggcaccagcatcacgatcttcagctctcagtgtggccagagccagggttggggtactgaagctggggcctgggcggggcagacgtaggcgcagaggactggtggggaaggtgggtgcatggtcattgacatcgcgcaccgtgatggtgacagacactgtggtgcttaggggcccagcagctgcaccatccactgcactcacagaaaaggtgtagctgggacactgttctctgtccaaggctgcagctgtgcgcagttctccagagctgggctccagcaggaaggctcctgctgtaccggcgcccaggtagtaggtcacatggccattagctccagcatcagggtcatgagcctgtagctgcagcagcagggtccctgcaggcacatcctccggcacctccaccgagtaggcaggcacaggaaaggctggagcatggtcattggcatccagcactgtcactgtcaaaagcagcgtggcactgagagctggctggcctccatcccgggcctctatcctcagctggaaagctggctccacttctctgtctagtggccgcatggtgccaaactctccagaagcaaggtctaggacaaaggctcctgatgggtccccatctaggatgcggtactgcaactgcccattggctcccacatctggatcagaggcccgaagcatggtaagggtctgggggtcctggccctcaggcacctccagagagagatgggcactcccaaaggttggtgcatggtcattctcatcctccacagccactcgaacagtgacatgcgttaactgaggaggtgagcccctgtcctgggcatacactgtcaggttgatctcctcctgttcctctcgatccagggcccgaagagtcgtgagaacaccagtgtcaggatccagagaaaagctttcgctagagacgcctccataagtcacttgcccgttggcccccacgtcggggtcggttgctcgcagggtgagcagagatgtgccaggagggttgttctcacgcaagaggacgctgtactcctgctgctggaaagtaggcgcctcgtcgttgacgtcagcgacactgacggtcaggacctgcgtggccgagcgcggcggggagccgtggtctgaggccaccactgtcagtacgtgctcagctcgttgttcgcggtccaacggccgcaccacggacagcgctccagtgcttgagtgcagccggaagtggccgtccccgccagatgccagccgataggacacgcgtgcagcctcgcccagatccgggtcccgggctaccacgtgcagggccgcgggcccaggcggctggtcctctgggaggcgcacgcgtgacggcgaggcgaagacaggcgcgttgtcattctcatccgtgacgaagacgcgcgctgaaacgcgcgctgcacgacggcggctggcgttggcgggccggtcggtggcttccaccagcagcagcagcgcgggagtggtctctcggtccaggccgcgcggagcgctgagcgccccggtgcgcgcgtccaggcgaagcgccggcacgggcggctcctggcgcagcaggcggtagcgcacgtcgctattggggccggggccgtcggcgtccgacgcgcggaaagtgtacagcgctgcgccgggctccgggttctctggcagcgccagcgccagcgggtcgcgcgcaaaggcgggcgcatgctcattctcgtcctgcacttgcacctgcactcgcagcagccgcgcgcccgcgcctcccggcccctcagcgcgtaccgtaagcgcgcgccacggcgggccagcttcgaagtccaggggccgcgccaggtacaagcgccctgaggccgcatccagcgcgaaggtgccctcgggatcggcaccgcccaccagtgtgtaggtgagtgcacccacacccgcgggctctggcgctgccaccgagcccaacagagagccgggccgcagtccctcagctgctgtcaccgtcagcacgacaggcactggtgccgctgggtcccgctctgcgagatctgggggcggctcggccaagcgagctgagggaagcacctgcaccagcagctggaggctggcacttcgaggagggctgccttggtcatgagcactcagtgtcagcacatagtggggccgctctgctcggatcaggggagctgcagtgagcagctcccctgagtgagggtgcagagagaaaagctctgagccaggaccagttagcgtgtacaagatggtcccattctccccctcatctggatccttcgcctgcagagtcgtcaccagtgttcccggaggcacgcggtctggtacctgtatagggaggcccccaccagcagctcctgaagcctgcaggaacgtggggctgttgtcgttgaggtcaagcactgcaacatgcacagtgcctgtggtgctgcggggtgggctccctccatcctgcacctgcaccaggagctgatagctgctctgctgctcacggtccagggtttggagtgtggtcacttctccagtctgggggtggatgcggaaggccttgctgtcttcagacagctgttgcaggctgtaggtcagacgtccattgggtcctgagtctcggtcagtggcaaagactcggcccacgctggtccctgggggctggttctcagccacagccaggaaggtgggatcctcagacaagcggggactgtgttcattctggttgaggatgctgaccctcacggtggctgtgcctgtctgctgccccaactcagctttggacccagacactgccattaccttcagtatgtacaattcctgggcctcacggtctagtgctgcccgcacccatagccacccactctgtggctccaggccaaaggggctacttgctccctctgctgcaaggtgataggtgatagggcccccatctggtgcttgggcctgcacttgcaggacctgagttccagcagtggtgcctgagggcaggtccacacggtaggtagggctgttgaatcggggagccagcccacgggttcccacatcctgtaccaccacccgtagtcgaaagtggctggtgcgtggtggggagcccccatcccgggcctccagctccagctcatgggctggccctcctgagggccccagaggcctcataagccgtacatggcctgtggtggggtccacggtgaaggctccaccacccccagcaagcagggtaaaggtgactcgactgttaacacctgagtcggggtcaagagcccgcagtgtatagatgggagtccctggggcagtgtttggtggtagcaataccgtgtcttcaggtgcaggaaaggcaggggagttgtcattcacatcatccagcagcacacgcacccgagctacagcgaaagctgggggcactccactgcctgctcgcacctccagctccaacactggtcccagtagctcccggtccagagggcgaagtgtttgcaacagtcctgataccgcatctagggagaagagtcctcggggatccccacctgatagggaaagggtcacaggtgccaagcgacctggtgggttgtgtgcctggactatgcccacactggtgcctggtgccacatcctctggcacagaaaaaacatactgtagttgctcaaatatgggtggtgtgggggttccaggcacaatgctgatgtccactcgggcactgggttctgcctgtaggccacctccgtcctcagccccgatctccagctgcaccacagaattggcccgtctggccaagggccaggctactgtcaacagccctgattgctcatccaaggtaaaaagtggggggctgttgccagccaggatatggtaggagagtcgcccatgggatccctggtcagggtcatgggcacgcaacctcagcacagctgtgcctggtggactctgggcacttatactggcagcatactcccgtggataaaactgaggagggttgtcattctcgtctgacagaaacaccttcacatataccatggacttgaggcctcccccatccacagctgtcactgtgaagtcaaagcttgagggcccctggtcacggtccagggtccgggttgtgcacacatcaccgctgtgggcatcaatgcggaatgggggagatccggaggacccaagtccagcacccaaggaataggagaggaggccaaatgggccactatccgcgtctgtggctgtcacctgcaggaagcaagttccaggctgggtgccctcaggcagtgaggcattgtagaaagtcctctggaattggggctcattatcattcacatcttgcagggccacgctaactgtggcagaggaggctagagggggcaggccaccatctgtggccaccacaatcagctgtggctgaggttccaactcatagtccagtgaggcagccgtagtgataatgcctgaggtggggtcaatggagaaccagtgggtgtgggcgccaggggctaggctataagtgacctgaccattggtgccttggtcaggatcccgagcagtcacccgcactacaaagctgccaggcagcgcaacctcaggcaggggctcaggtcggtagagctggcggtcaaaggcaggtgcattgtcgttgacatcagtgacgtgcagcacaaaggcagcctcagcccgcagtggaggtgagcctgagtctgtggctgtaaccctcaagttataggcatccctctcctctcgatccagccgccgagccacacacaccagatagatgacgctgtcttgggtgcttagggcaaagtggccctctccaccttccagggacacattgacatgggcaaagtcaccatcatctgggtctgacacagagatgcgagcaacgagctgtccaggtggggcggcctcagacacttggggggagccatctgcactgagaaagatgacagtcatggagggctgattgtcattggcatctcgcacatgcacagtcacaaaggccgagcccagctcagggtgagccccaccatctcgtgcttgcaccaccagttcatggacccgccgctgctcaaagtccagtggccgctctaactgcagcagccccgtgtgtgcgtcgatggagaagggtccatcaccctcgctctgcctccggttgatctcgtaagtcacagccccattgacaccagcatcggcatcagatgcgaacacctgcaagacaggactgccaggggccaggctctcagacaccacagcatggtagcggctctgattgaaagccggggcatggtcattgatgtccagcagtgtcacgtccagcagggcctgggccctccgggggggtgaaccaccatcataggcctccagctgtagcatatagtgtgagcggttctctcggtccagttccccagtaactaccagctcaggtactggagtcccatctggaccggggcgtgtctccagccggaaggtctctccagccccatcaccagatagcgcatagccctgggttcccagacgcccagcatctgcatcacgagcaggctccagtgggtagcgggtgccaaaagctgtatgctcaggtacctgcagggcagcccgagcctgtgggaaggctggagcatggtcgttgatgtcagccactcgcactgtaacttctacggtggcaccatcaggagtgactgcagtgaagcggtagcggtcccgctgctcacggtccaagacacgggctgtacggacgaccccactgtgttcgtcaatggccaggtctgtgcccacgccgctgccctcttgggcagagatgaagtacatgagaggagctgccgtgcctgccggaagccccgcactgatgtcgccaatcagtgtacccgctggctgctcctcatcaatctgcaagtccaggctcccagcctgaccccaggcacctggcaccccagcccccagcagcagcagcagcagcagcagcaatggtagcaggaggtggggcctggggctcttcatgccagggcaggaaggcacaatgcccagctccttctgcatgacaagggtagtccagctgtgccttgggctccagctccaggccaggctctgggcccagcttgacctcagactttgggtcaggtcccactggggccctggctccagctcaggctccctgacctccgcgcgacgcgggctccctcgcccggtgctggggcgccgtccggccgcggtcagccccccgggcagcgcccgctcgcgcggggcctgaggccgcgcatcgtccgcagtcgctgtctccgaggcccgcgatcccctccgggcagccgccgtcggtccgcgcgcccttggccgtcgatcggtccgtccgctgacgcccgggcgccgcctcctgcacagccgccccgccgaggatgcgagctccgct

SEQ ID NO: 16342 - RNA, 1634 nt, Homo sapiens
  source 1..1634: mol_type = other RNA
gggtcccggggaggggggaagctgggggtttcttttgcctgcagggtgtggggaggagcagaggagggccaagaaagggagaaggaaacagaggccacagaggcctggctggaggtatcctgctgccccctgccctgtcctggagctgcccttggcctcctgtgccctctaccggtgcacgcctgtgtgggcccagcccccatctgtctggtctggccctgagaggctcgggcaccagctgcatcatttctctttcttctccagccccttcgatgctgatgcctctgttccctctttggattctgtcactgccgctggatccttaggatttgactcctcataaatggcgctgggattctgcgggcgccggcggcgagggccagctagcttctgctgcatggagtcggccaggctggctggggagcccgagactgtggggaagtgggtgagcctcggggtatgaggcaggatttccgccgaggactcgtagctgaacatctctgtcacttctcccttggccagcgccaccaggacaggaaaaccgatgcaggcggggaccaggtataggagggcaggctgagcatgcttgaagatgtgcatgatgaagatggtaaggcccaggccgaagatgtaggctgcaaagctggtgtagaagtaggtgtgggtattcttcttcaagctgatgtcaaagcgcagcagcaaggcaatgaagatccctggaatgacgacatctccaagtcccagcatggcaaagttgtttgcttcgaggcctttctccagcagatcctggggaaacaccaattttattggtgcctcgaaggacttggccactgtcaccatcacattggtgccaaatacccagaagacatcgtagatgaagagtccgcccagcaggatgcagccagtgctgacattgttgaggtgcaggagctctactccattaagggagaaggccaggccaaaaaggttgttggcaatccagtgcttcctcagcaggtaccagacgccaacgatgctgctcaggcccaggcacaccaggtccttggtgtcaaattcataattgatgatctcttccttgttttccccagaaccctgtgtgaagagcagctggtactgtcgatttggaaagctggctggaaaaaacttattcatgaaggggctgatggtgtgggacagggccaggattcccagcacgaagaaatacatggacagcaggaggttgatgtactcctgggagaatattttgaaaaagaggtagagccccaagagtgtgcagctggcgatgatggggaagcgggcggcatcccggctggtgattgtttcaggcatgtctgaagcattcttgccgcgggcgcagcgtacggagcgcagggcgccgaagaagatgggcagcagcgccatgagcaggaggctgccgtaggccagcgcgatgccctcgggcgtggaaggcggccgcgtagtgctgttggtggggccgcctgcctcggcactgccgttatgcggatcgctgagggccgagtccatggcgagggtgcgttcgggatccgactccagctccggttgctgcagcagggacgcaggcggagacaccggctctgcagggaaagccacgttcccctaaggcaacaggaagt

SEQ ID NO: 16343 - RNA, 1487 nt, Homo sapiens
  source 1..1487: mol_type = other RNA
gggtcccggggaggggggaagctgggggtttcttttgcctgcagggtgtggggaggagcagaggagggccaagaaagggagaaggaaacagaggccacagaggcctggctggaggtatcctgctgccccctgccctgtcctggagctgcccttggcctcctgtgccctctaccggtgcacgcctgtgtgggcccagcccccatctgtctggtctggccctgagaggctcgggcaccagctgcatcatttctctttcttctccagccccttcgatgctgatgcctctgttccctctttggattctgtcactgccgctggatccttaggatttgactcctcataactgaacatctctgtcacttctcccttggccagcgccaccaggacaggaaaaccgatgcaggcggggaccaggtataggagggcaggctgagcatgcttgaagatgtgcatgatgaagatggtaaggcccaggccgaagatgtaggctgcaaagctggtgtagaagtaggtgtgggtattcttcttcaagctgatgtcaaagcgcagcagcaaggcaatgaagatccctggaatgacgacatctccaagtcccagcatggcaaagttgtttgcttcgaggcctttctccagcagatcctggggaaacaccaattttattggtgcctcgaaggacttggccactgtcaccatcacattggtgccaaatacccagaagacatcgtagatgaagagtccgcccagcaggatgcagccagtgctgacattgttgaggtgcaggagctctactccattaagggagaaggccaggccaaaaaggttgttggcaatccagtgcttcctcagcaggtaccagacgccaacgatgctgctcaggcccaggcacaccaggtccttggtgtcaaattcataattgatgatctcttccttgttttccccagaaccctgtgtgaagagcagctggtactgtcgatttggaaagctggctggaaaaaacttattcatgaaggggctgatggtgtgggacagggccaggattcccagcacgaagaaatacatggacagcaggaggttgatgtactcctgggagaatattttgaaaaagaggtagagccccaagagtgtgcagctggcgatgatggggaagcgggcggcatcccggctggtgattgtttcaggcatgtctgaagcattcttgccgcgggcgcagcgtacggagcgcagggcgccgaagaagatgggcagcagcgccatgagcaggaggctgccgtaggccagcgcgatgccctcgggcgtggaaggcggccgcgtagtgctgttggtggggccgcctgcctcggcactgccgttatgcggatcgctgagggccgagtccatggcgagggtgcgttcgggatccgactccagctccggttgctgcagcagggacgcaggcggagacaccggctctgcagggaaagccacgttcccctaaggcaacaggaagt

SEQ ID NO: 16344 - RNA, 1690 nt, Homo sapiens
  source 1..1690: mol_type = other RNA
gggtcccggggaggggggaagctgggggtttcttttgcctgcagggtgtggggaggagcagaggagggccaagaaagggagaaggaaacagaggccacagaggcctggctggaggtatcctgctgccccctgccctgtcctggagctgcccttggcctcctgtgccctctaccggtgcacgcctgtgtgggcccagcccccatctgtctggtctggccctgagaggctcgggcaccagctgcatcatttctctttcttctccagccccttcgatgctgatgcctctgttccctctttggattctgtcactgccgctggatccttaggatttgactcctcataacttgggccccggggcagtagggggaagcgggcaggtgggcacccgctgggcattacatggcgctgggattctgcgggcgccggcggcgagggccagctagcttctgctgcatggagtcggccaggctggctggggagcccgagactgtggggaagtgggtgagcctcggggtatgaggcaggatttccgccgaggactcgtagctgaacatctctgtcacttctcccttggccagcgccaccaggacaggaaaaccgatgcaggcggggaccaggtataggagggcaggctgagcatgcttgaagatgtgcatgatgaagatggtaaggcccaggccgaagatgtaggctgcaaagctggtgtagaagtaggtgtgggtattcttcttcaagctgatgtcaaagcgcagcagcaaggcaatgaagatccctggaatgacgacatctccaagtcccagcatggcaaagttgtttgcttcgaggcctttctccagcagatcctggggaaacaccaattttattggtgcctcgaaggacttggccactgtcaccatcacattggtgccaaatacccagaagacatcgtagatgaagagtccgcccagcaggatgcagccagtgctgacattgttgaggtgcaggagctctactccattaagggagaaggccaggccaaaaaggttgttggcaatccagtgcttcctcagcaggtaccagacgccaacgatgctgctcaggcccaggcacaccaggtccttggtgtcaaattcataattgatgatctcttccttgttttccccagaaccctgtgtgaagagcagctggtactgtcgatttggaaagctggctggaaaaaacttattcatgaaggggctgatggtgtgggacagggccaggattcccagcacgaagaaatacatggacagcaggaggttgatgtactcctgggagaatattttgaaaaagaggtagagccccaagagtgtgcagctggcgatgatggggaagcgggcggcatcccggctggtgattgtttcaggcatgtctgaagcattcttgccgcgggcgcagcgtacggagcgcagggcgccgaagaagatgggcagcagcgccatgagcaggaggctgccgtaggccagcgcgatgccctcgggcgtggaaggcggccgcgtagtgctgttggtggggccgcctgcctcggcactgccgttatgcggatcgctgagggccgagtccatggcgagggtgcgttcgggatccgactccagctccggttgctgcagcagggacgcaggcggagacaccggctctgcagggaaagccacgttcccctaaggcaacaggaagt

SEQ ID NO: 16345 - RNA, 1081 nt, Homo sapiens
  source 1..1081: mol_type = other RNA
gggtcccggggaggggggcagggtgggggacgaggaggcggagaggagtctgtgtgcctgggcggcgggcgaggactcccccatgctcgccaggagcgcgggccaggagggctcctgctgccgccgctgctgctgctgctgctgccgctgcctctgctgctgctgctgctgctgctgctgccgctgctgctgctggtgctccttgtcccgggcccgggtcagcttggcctcggcgcagaaccacaagtgatcagagagcaggactgtgaaaaacaagagagatgccagagacagtcgccatttctgagccctctcggaatcgatgaacggtttctcgttctctcggggtgctgccaaccagatttttaagccgtcgtcatactgccgacacatccaagcacccctggtcatattttgggaacgcacagccctggccgactccaccgtgagggcgcctgtgccggtgtcaccacaatatgcattgacttaaagggtttaatttccttatcccctcctcccgtttcttctctctcctctctctctttctctctcttcccctctccctctctcctctctctctctctccctctccctctcttttatctctctctgtctcttttgcctacataaatattaccaggctttgaaggaaggtctgacttgcttcctaatcatcagccgaccccatcctctgtagagtgggaaacaataatggagagagagagagagagagagacggaggaggctggtgctggtggccggcggcgaggctgggtgcagggggcgatggtggaggtgacagggtggctggcgcggctccggtcacccaggcattgtcagcgcgcgggtccccatggccccgcggagcccagcccgctctcccctgccaggggcatgccgcgcctccgctgcccactgacggcgcccggagcgcctcccctcctcctcctcctcctcctcttcttctcctcctcttcctcctccttcctttccttctccttcttcttctcctccgcctcccgctcctgctccgcgctggctctcccagagtccggagcctgggctgcctccggcggggcgc

SEQ ID NO: 16346 - RNA, 1311 nt, Homo sapiens
  source 1..1311: mol_type = other RNA
gggtcccggggaggggggcagggtgggggacgaggaggcggagaggagtctgtgtgcctgggcggcgggcgaggactcccccatgctcgccaggagcgcgggccaggagggctcctgctgccgccgctgctgctgctgctgctgccgctgcctctgctgctgctgctgctgctgctgctgccgctgctgctgctggtgctccttgtcccgggcccgggtcagcttggcctcggcgcagaaccacaagtgatcagagagcaggactgtgaaaaacaagagagatgccagagacagtcgccatttctgagccctctcggaatcgatgaacggtttctcgttctctcggggtgctgccaaccagatttttaagccgtcgtcatactgccgacacatccaagcacccctggtcatattttgggaacgcacagccctggccgactccaccgtgagggcgcctgtgccggtgtcaccacaatatgcattgacttaaagggtttaatttccttatcccctcctcccgtttcttctctctcctctctctctttctctctcttcccctctccctctctcctctctctctctctccctctccctctcttttatctctctctgtctcttttgcctacataaatattaccaggctttgaaggaaggtctgacttgcttcctaatcatcagccgaccccatcctctgtagagtgggaaacaataatggagagagagagagagagagagacggaggaggctggtgctggtggccggcggcgaggctgggtgcagggggcgatggtggaggtgacagggtggctggcgcggctccggtcacccaggcattgtcagcgcgcgggtccccatggccccgcggagcccagcccgctctcccctgccaggggcatgccgcgcctccgctgcccactgacggcgcccggagcgcctcccctcctcctcctcctcctcctcttcttctcctcctcttcctcctccttcctttccttctccttcttcttctcctccgcctcccgctcctgctccgcgctggctctcccagagtccggagcctgggctgcctccggcggggcgctccctcccccccaccccccaccccgcgctctaagtgctgccgccgccgccgccgccgccgccgctgccgcagggccgcccgcgggcgccgccgccggggctccgactgctgacgccgcctcccgcggagctccgggccgaatcgcctgggctgggcctcccgagagccacagtcatcttcagtccgcgggctaagttgccgccatcttcgtcctggagaaacactttttt

SEQ ID NO: 16347 - RNA, 393 nt, Homo sapiens
  source 1..393: mol_type = other RNA
gggtcccggggaggggggggtcgctgtaacctgcccccctcccctgggcccgcccctggactgcgaccccctgccctacggctgcgaggcgagcggagggggaggtgaaggaagctgctccggccccgccccccccagcccgcgcgcacccccgacctctccccctcccccaagcgcgcgaccctcgggagatagggatttaaataaaatttgaataaatccccctcctcaagcgggagggtggaaggaaaggatagagggggagagggaaaggggaagggggcagttggggtgtctcagcccccctggtcccccagccccgcgctgctacggcccggggccctggccgcctctctcatccctcctcagctccttcctccttcctcctctctt

SEQ ID NO: 16348 - RNA, 191 nt, Homo sapiens
  source 1..191: mol_type = other RNA
ggtctaggcccggtgagagactccacacagcggagaactgccattctttcctgggcatcccggggatcccagagccggcccaggtaccagcaggtgggccgcctactgcgcacgcgcgggtttgcgggcagccgcctgggctgtgggagcagccgggacagagctctcccgcctctccaccgccccacccc

SEQ ID NO: 16349 - RNA, 1766 nt, Homo sapiens
  source 1..1766: mol_type = other RNA
ggtggatattccttctatgttccctttagggccattttatccatgtattctttagagaattcttacctttagagaatgttatcaatatatagtagagatgcaatgccaggaggcacaccccaaaattatggaaccaagggaaatgaagcaggttcagagaatccttcagagcatgtgctagaagcagtcagtgctccctgaatacctgctcttcccttaatttgctagctttccttgaagttggatgaacccatgtcactagttctgagcaatggtcttcaagcagaagtaaagccaagtgaaaaaatgtacctggaagacagagtgttcaacgatatcagatgccacagatagatcaaataaggtgagaattgagaattgattatggggtttggtaaaatggaggtcatcatcgactttgaaaagaatagtttttctatagaaattcattacgagcatcactgaatcagactataaggaactacttcactagtgagtatagaacttaggtctatacaagttagtcaattattgacatggagttagagagcctagatccttccccactcaaacctatgctgttctctcacctaacccaccagaagcctggtttgctttccttgttccattacacatccatatacatataggtcacattgtcaaaattttaattatcggcccaaattctttactctcctctagtagtgctacacatctgtacccttgccatggtcttatggatgtgtaatgtactactgagccccttaactatgtggttggtcatattatttacattggtcaattggacattagcaaaaacaacctaggtggaaaaactgaaatttgcttgagcaattgcactttccctctgcaagtctacatagccctgagtcagtccacatacccaggatagttcactggtcccatagagacacccaaagctaaccacagcctggaacgaagtctagtctacatgagccaaacttcagtcaacctgcagaagcacaagcgagaaagaaatgacttttttgttagaagccactgaattttgcagcggctggtatatagcattattgtgaatatagctgattaagacacaagttgtggtagaaatatttcaaatgtcctttaaaaataagtaacatagttcttcctgaactcttctttaattacaaacttcagattgatcccaaaatgccatgaagccactccacccaatacccacaccacagtaaagttggtcactctcctcttaagaattcagtctttaaggactggaagggacctgagtaatcatgcccagccacctctttttacctctgagaacacccaggaggtgaaatgacatgtcaaatatcacattactaatcactgagaacagtgattggaaactagatttctcacggtgttttcaggcctatttgtactgtgtcacactgcttgtcttaattccaaattgaggactctcaggttgaagctacagtcagaaacaagagatctagaattaacattataaacactcattctcttgtcatctactgtaacatctttctctttgtttaagcccctttctctccagtgcctgaactaccaccactaacacacatacacacacacacagagttttggatttggtctttagtctttgctttgattatgattatgcatccttcaaaaatctctgttccatcaataattagcatatatgtttaaaatatttcgctggaatcatagatgacacaaactactggaaaagcattccatgc

SEQ ID NO: 16350 - RNA, 2030 nt, Homo sapiens
  source 1..2030: mol_type = other RNA
ggtggcccggccgtgcctgaggtttctccccgagccgccgcctctgcgggctcccgggtgcccttgccctcgcggtccccggccctcgcccgtctgtgccctcttccccgcccgccgcccgccgatcctcttcttccccccgagcggctcaccggcttcacgtccgttggtggccccgcctgggaccgaacccggcaccgcctcgtggggcgccgccgccggccactgatcggcccggcgtccgcgtcccccggcgcgcgccttggggaccgggtcggtggcgccccgcgtggggcccggtgggcttcccggagggttccgggggtcggcctgcggcgcgtgcgggggaggagacggttccgggggaccggccgcgactgcggcggcggtggtgggggcagccgcggggatcgccgagggccggtcggccgccccgggtgccgcgcggtgccgccggcggcggtgaggccccgcgcgtgtgtcccggccgcggtcggccgcgctcgaggggtccccgtggcgtccccttccccgccggccgcctttctcgcgccttccccgtcgccccggcctcgcccgtggtctctcgtcttctcccggcccgctcttccgaaccgggtcggcgcgtcccccgggtgcgcctcgcttcccgggcctgccgcggcccttccccgaggcgtccgtcccgggcgtcggcgtcggggagagcccgtcctccccgcgtggcgtcgccccgttcggcgcgcgcgtgcgcccgagcgcggcccggtggtccctgccggacaggcgttcgtgcgacgtgtggcgtgggtcgacctccgccttgccggtcgctcgccctttccccgggtcggggggtggggcccgggccggggcctcggccccggtcgcggtcccccgtcccgggcgggggcgggcgcgccggccggcctcggtcggccctcccttggccgtcgtgtggcgtgtgccacccctgcgcccgcgcccgccggcggggctcggagccgggcttcggccgggccccgggccctcgaccggaccggtgcgcgggcgctgcggccgcacggcgcgactgtccccgggccgggcaccgcggtccgcctctcgctcgccgcccggacgtcggggccgccccgcggggcgggcggagcgccgtccccgcctcgccgccgcccgcgggcgccggccgcgcgcgcgcgcgcgtggccgccggtccctcccggccgccgggcgcgggtcgggccgtccgcctcctcgcgggcgggcgcgacgaagaagcgtcgcgggtctgtggcgcggggccccggtggtcgtgtcgcgtggggggcgggtggttggggcgtccggttcgccgcgccccgccccggccccaccggtcccggccgccgcccccgcgcccgctcgctccctcccgtccgcccgtccgcggcccgtccgtccgtccgtcgtcctcctcgcttgcggggcgccgggcccgtcctcgcgaggccccccggccggccgtccggccgcgtcggggcctcgccgcgctctaccttacctacctggttgatcggttctcggcggcgtcgcggcgggtctgggggggtctcggtgccctcctccccgccggggcccgtcgtccggccccgccgcgccggctccccgtcttcggggccggccggattcccgtcgcctccgccgcgccgctccgcgccgccgggcacggccccgctcgctctccccggccttcccgctagggcgtctcgagggtcgggggccggacgccggtcccctcccccgcctcctcgtccgcccccccgccgtccaggtacccggcggccgtcgcgcgcctgccgcgcgtgtggcgtgcgccccgcgccgtgggggcgggaacccccgggcgcctgtggggtggtgtccgcgctcgcccccgcgtgggcggcgcgcgcctccccgtggtgtgaaaccttccgacccctctccggagtccggtcccgtttgctgtctcgtctggccggcctgaggcaaccccctctcctattgatcat

SEQ ID NO: 16351 - RNA, 148 nt, Homo sapiens
  source 1..148: mol_type = other RNA
ggttccctctccaaatgtgtctaggataccttagagcttgatctcataaggactgctgtcctctctgctcactgccttgtcctcacaggccaatttcgtcacacgtgtgttacaggtgactccaataggaaatccagcttctctttgg

SEQ ID NO: 16352 - RNA, 72 nt, Homo sapiens
  source 1..72: mol_type = other RNA
ggttccctctccaaatgtgtcttgatcccccaccccaagacacatttggagagggaccctcccaactcagat

SEQ ID NO: 16353 - RNA, 135 nt, Homo sapiens
  source 1..135: mol_type = other RNA
ggttccctctccaaatgtgtcttgatcccccaccccaagacacatttggagagggaccctcccaactcagataaactgtggagagtgtaggagataggaaatggactgagaacttcctggtcccaccagagaagc

SEQ ID NO: 16354 - RNA, 68 nt, Homo sapiens
  source 1..68: mol_type = other RNA
ggttccctctccaaatgtgtcttggggtgggggatcaagacacatttggagagggaacctcccaactc

SEQ ID NO: 16355 - RNA, 319 nt, Homo sapiens
  source 1..319: mol_type = other RNA
gtaagcaggggctctgggtgaaacaaaggttgagggctgaggggatggggtctcgctgaccccatccttgactctgccaggaggggccctccaagttttccaccctggagatgaaccccaagagcccccagaagaggccaacggagatgatgagagtgcctgaggctggggaagggcaagggagctgccccaggagtggggagaggggccccccggccctttcctcctgtggccacaatgcctgcaggccccattagaggtggccttctctggactgtggcaaggctgtgcctggaccagctggtgtcccagatggtgg

SEQ ID NO: 16356 - RNA, 641 nt, Homo sapiens
  source 1..641: mol_type = other RNA
gtagaggagatggcgcagggcacgatgcccaggctctggggtgagctgtccttcccgatcatggtgtacgacttgcccaggctcatgtggccaaaggaaaaaatgcagccatcagccccactgaccaccgactggagcacgtcggccacggtccccgagcagacttcggcctgctcggagtcctgggggaagacggcatcgaaggcaaacatcttgggaactgcagcagtggcggctcgccgggggcctgcgctgcctgggggaccggcggcgggatcgtagaggatcacctgcttcttccgagggtccaccttcaggaaggacatggcctcggccgagcgctgggccccctgtgcgggccagatccgcagcataaccttcaccttcccgatgctgccagggttgtccttggtcttggaggcggccctgagcaggcaggggggcgccgggggcggccacagctgcaggaccccgctgaagtcggtggggtaggtggaggtgccgcgggtggctggaggcggtggcgggtggggcttcttcctcttggaggccaggctgagcttctgcatagcccaggcacgccggcgggaggaagctgttgacccgcgagacactccacatgccctccaggcactgctggg

SEQ ID NO: 16357 - RNA, 1632 nt, Homo sapiens
  source 1..1632: mol_type = other RNA
gtagaggagatggcgcagggcacgatgcccaggctctggggtgagctgtccttcccgatcatggtgtacgacttgcccaggctcatgtggccaaaggaaaaaatgcagccatcagccccactgaccaccgactggagcacgtcggccacggtccccgagcagacttcggcctgctcggagtcctgggggaagacggcatcgaaggcaaacatcttgggaactgcagcagtggcggctcgccgggggcctgcgctgcctgggggaccggcggcgggatcgtagaggatcacctgcttcttccgagggtccaccttcaggaaggacatggcctcggccgagcgctgggccccctgtgcgggccagatccgcagcataaccttcaccttcccgatgctgccagggttgtccttggtcttggaggcggccctgagcaggcaggggggcgccgggggcggccacagctgcaggaccccgctgaagtcggtggggtaggtggaggtgccgcgggtggctggaggcggtggcgggtggggcttcttcctcttggaggccaggctgagcttctgcatagcccttatgaagaaggaggctgcagctgaggggcctgtggagccccccaccgagcccggggtgggggtgaccagggctgacgtgcagactccaccacggccccaggccttcgacaagccatcagggccggccacgggggggcattctcggaccgtgtctgccaccgccacggccgccaccgctgcctcggccaggcacgccggcgggaggaagctgttgacccgcgagacactccacatgccctccaggcactgctgggcctggatggtgaccgtgctcagcgcccctccaagacccgcaggtgctacagacacctggacactgggcccgggggaccaggccagccccttggtcctgtctggcccagctcgtcctggctgcctccctgcaggacccgctggtcctggcgtgtccctcgagctggtcgtggtgctggggggtgcgaggctggggcctccatggggggcgtcaaggtcctcatggctggcaggggcctgcagcaggtgcatggcctcccgtgtgagctgctgcaggtgtgtggcgcagacgtcacagcggcgctcggcctctgggcgacaggctggcagggccccaggtgctggtagcttgtcgagaagcagggcagagaggcaaggatcccggagggtggtcccgggcccgctgaccagcttccacgcctgtcgcttgagctccaccagcttcgtgtggcagtggcggcaccagccgcctccgccggccgagtggccctgctctgggccggccccggcgccttcgggagcagggcggctgccgcatgggtcctggtcgggcccggcgggtagcctctttcggggggacacctccagcagcggcggcggctcgcgggccgggccgccctcggccaccgcgggctgcgcagcgcacagagggacgccgcggccgaccatggccggggcgcgggaagagcccggcaggcgctcccggccacgctggctctccgggggcgccgcggctacgtgatccggccccgaggcgcccccatggcccggcccagccgctcggaagttcgcagagcctgcgagt

SEQ ID NO: 16358 - RNA, 4839 nt, Homo sapiens
  source 1..4839: mol_type = other RNA
gtagattctccttctatgagtaagagagtgggaaaagtcaaaacgcagctccatggagataacgtctcatggtgagtcactgctttgctgaaatgattcttgtactctctgctacacgacaggaaaaatgttaacgctgctttgccattaaagcaagcatttcatttcctgcttgaaatgccaactgagcaagatttccattcacttctagaaaaagacaccgcagcatattgtgcttcttcaacactgaacctctcttaattttcagtgttttggtaaagataaggtcattattgctcattagcaatttatctgctttttaaaaattcatcttctctaaacaaacgaaaaggacagaaggtgggaagcacaacaccaagaattcaaaaaaacaatggtggtggtgtggaaaattttcagtgaaatcaataccagttcaataaatcctttgaacaagttctcatttgtgaagaacccaacaggagttttaattaaatccaggatattaagagtaagattaaagttttatagctagatgaaaaatataatacagttatctgtctttgatccagatatgatagaacattatttttgaaatatctcacatacactataaaatagcaatttccagggtggaaatggaactcattataaaacgtcagagagtactgctctaattcgacacatttcttttctgtctcttcctcaagtagaaaatagcacttgagctggtgatttttatttctccttttggcacatgtgcccacacactgccatcatttctcatcaggttactgagactatgtgagcttttcagtgtacttagggtaatttctagatatttctttgtgctgcctttgtgtatatgatccactacacatctgagttttcatctcgcagaagggcatccagactgcaatgtcttctaagctctaagctggctacagactgtggctgagcagtagaagatgcgtagccctctctaaccaacgcggaagaacctgagggtcatctggaaaccttagcagtggaaatgctaggtttggcccttgggcttttggctagcccagggtcaagtgttttttttttcactttttttttgttattctaaataagatacatagcaattaaaatagagaacaaataatggatgtttcctcaccatttgtttcatttcaaataaatataaacacatttacagcaaaagtatatggacattttctctagtttggcaaaaaaaaaaaaaaaggtcagcacatcatcagttacaaatgttaagtggtcaactagaaatctgtgtcctaagaaatataaaatacaacaaagactggtacacagaaagattacatttaactccataaaaaagctacttcagttctcacttgcattttgaaggaaaaaaatgtgtatcttccattttagactgaagcattttggtcctcatgtgtagctggctgatgaactacacacacacacacatatatatatatatacacacgcacacatatatgtgtgcatgtgtatgtgcataatttttaaagagtctcattcttctttttgtacagcggttccaggtgtggaacggggtccatttgacctagaagcattttcatctacagcaagtacacaggcccctttggccagcaactcctcaactaccacctttaagccattgcgcgcagcgacgtggaggggtgtctgcagtgcattatttttttcattaataaggctctcgtcttgtatcttgtcaagtattaacaaggcacatttttcatgacctttactacaagccaaatgtaagggtgtattcaagtccttatcctttacagtcagatcagcctgggcactgttcaccaaaatatccacagcgcctgcctgcccattctcagcagccatcatcagtgctgttttccctgaattatctactgcgttcactggagcactgtgtctcagaagaagctgcaagcactccacatgatcagcaaatgctgccgcatgaaggggtgtcctgcctttgtcatctctacaactgacgatactggaatctatggccccaagcagcaatgatgcacaattcccatgatcattgattattgcacagtgcagtggagtaaagggattaccgataaatttgcgaaaacatttttgctccaaaagtacctctatacagttttcattaccattgtaacaagcccagtgcagcggcgtgtagccttggttatctttgaaacaacagtcctcctcagaaagagccatttggagcagctcgctcagccacgtggcgtggccacgagcagctgcatagtgcaagggcgtcctccctctggaatctttacagagaattgacacttcttgttccagcagcatttgcacacattcctcgtgtcctgtcataatccctctgtgtaaagctgtgcatcctaggatgtcaacagtgtctacgttggcttccttttcaagtaacaatgaaacagcgtcaatatgtccatatgctactgcaagcatcagtggtgtttgtcctttggcatctttcacatcgaccgcctccgggttgtctgcaatttctagcaacagccgtaaacacagtgtgtgaccattaattactgaggcatgaagtggggttcttttggttacattgtctttcacaaagatggatgcgccctgattgataagcgcttccacacattctgtgtgtcctttaaaggcagccagatccagagcagtgcggcctttctcatccctgatgtccaggtccaccaacgactgcagaaggacttccaaggcttgatggtgcccattgtaggcagctaagtggagtggactcttagtagcaccagaatctgattcttcaaatccactgtttgttctttccaaaagagattaatttggcatcttcattatgttgagtcttctaatccacgcatacagaatgtctctcctttttttttttttagatctctgatttctttcatcagcattttgtggtttcaacacacgtcttttggatctaggacaattccagacactgcctgtgcccataggcggcagcataatgtatgctattgtaaccttccttgtcccggatagatggatttgcatcattttgaagcagaaactctagacatagtgtggcttccttttccttcagctccctggctctttcaagttcttctgaattatcatgggcatttcctaagatagtcttatttctatccatgtctgatgcagcggcgtaatgcaaagctgtgcgtccccagtcatctgtttcattaacgttggcccctgtggtcactaatgtctcaatacagtggaaatgacaattcgcagctgcatagtgcaaaggggtcctcccacacttgtcctttttatggaaatctgctccgctgctctgcaagagttttatacattccacattacctcctgcagcagcagcatgaaggcacgttcttccaaatttatctggggtgtctatttcaaagcccgatgataacaactttctgcagcagtcagagtgagcatttagggcagctaaatgtaaagggaacatgctatggattccacacttggctgtgtcagctccgctggttattaaggtgttaatcaaaagctcatgaccgtatcttgcagccacatggagaggagtgttgccgtccttatccacacagtcaatttcacctccattctgaatgagggtctgtgaccgtgtgaaccttccatggacagctgtcatgtgcagtggacttttgccatctttactctgaatgttaacatctgccccgttgtttactaacaattcaagacacaaagcaccatgagtggaggcagcagcaaaatgcaaaggggtgaacccattattgtttggctggttcacgttagcaccgtagtcaatcaactcgttaaccacagcatcctgtccattgtagcaggcgatgtgaagcgctgtatttccatagacattgatttcatcaatctccacccccaggttcaggagatgcttgacaacattaatctgtccattggaggctgcagcatgcagaggggtataacccttcttatccttacaggtcacttctgcgccatggttaatgagcaatgctacaacatccaagtggcccatgtatgctgcccagtgcagagcacgccggtccttcttgtcaaatgcattgatatttgcccctttggccaagagtaaattgaccatctccacgtggccgttcagagccgcatggtgcaaggctgtgcgcccccctcggtcggagacattgacactgctcagcaggggaatgatcacttctgcacatttgacagccttgttggctgctgccacatgaagaggggtctgccagttcttgtcccttgcattgacatcagctgagtgcttaatcaaaacctgtactgcttcttcacttctggaagcaacagcccggtgcagtggagtcagccacatgttgtccttggcatttacacgagctcctgacaaaatcaggagttcaatgatctctgcatctcccagaaatgcggccacatgaagaggggttcgtttctcagaatccagagtattcacatcttcagttttatggatgagcatccggatctcctctggatcaccgctgaagattgcctgaaccaatggtggctggtcggtgagtttgagcactgccattcttccgctccttcgcgcgcacacacatgcaggtccccggcccgcagatgtcacgccgggagccggggaagcggaagggattgccaggagaagggaaaaaatctggctcccgaatttgacagccctccccctgctcctcctccgccgccgcctcctcccgccgagaggctgacact

SEQ ID NO: 16359 - RNA, 4703 nt, Homo sapiens
  source 1..4703: mol_type = other RNA
gtagattctccttctatgagtaagagagtgggaaaagtcaaaacgcagctccatggagataacgtctcatggtgagtcactgctttgctgaaatgattcttgtactctctgctacacgacaggaaaaatgttaacgctgctttgccattaaagcaagcatttcatttcctgcttgaaatgccaactgagcaagatttccattcacttctagaaaaagacaccgcagcatattgtgcttcttcaacactgaacctctcttaattttcagtgttttggtaaagataaggtcattattgctcattagcaatttatctgctttttaaaaattcatcttctctaaacaaacgaaaaggacagaaggtgggaagcacaacaccaagaattcaaaaaaacaatggtggtggtgtggaaaattttcagtgaaatcaataccagttcaataaatcctttgaacaagttctcatttgtgaagaacccaacaggagttttaattaaatccaggatattaagagtaagattaaagttttatagctagatgaaaaatataatacagttatctgtctttgatccagatatgatagaacattatttttgaaatatctcacatacactataaaatagcaatttccagggtggaaatggaactcattataaaacgtcagagagtactgctctaattcgacacatttcttttctgtctcttcctcaagtagaaaatagcacttgagctggtgatttttatttctccttttggcacatgtgcccacacactgccatcatttctcatcaggttactgagactatgtgagcttttcagtgtacttagggtaatttctagatatttctttgtgctgcctttgtgtatatgatccactacacatctgagttttcatctcgcagaagggcatccagactgcaatgtcttctaagctctaagctggctacagactgtggctgagcagtagaagatgcgtagccctctctaaccaacgcggaagaacctgagggtcatctggaaaccttagcagtggaaatgctaggtttggcccttgggcttttggctagcccagggtcaagtgttttttttttcactttttttttgttattctaaataagatacatagcaattaaaatagagaacaaataatggatgtttcctcaccatttgtttcatttcaaataaatataaacacatttacagcaaaagtatatggacattttctctagtttggcaaaaaaaaaaaaaaaggtcagcacatcatcagttacaaatgttaagtggtcaactagaaatctgtgtcctaagaaatataaaatacaacaaagactggtacacagaaagattacatttaactccataaaaaagctacttcagttctcacttgcattttgaaggaaaaaaatgtgtatcttccattttagactgaagcattttggtcctcatgtgtagctggctgatgaactacacacacacacacatatatatatatatacacacgcacacatatatgtgtgcatgtgtatgtgcataatttttaaagagtctcattcttctttttgtacagcggttccaggtgtggaacggggtccatttgacctagaagcattttcatctacagcaagtacacaggcccctttggccagcaactcctcaactaccacctttaagccattgcgcgcagcgacgtggaggggtgtctgcagtgcattatttttttcattaataaggctctcgtcttgtatcttgtcaagtattaacaaggcacatttttcatgacctttactacaagccaaatgtaagggtgtattcaagtccttatcctttacagtcagatcagcctgggcactgttcaccaaaatatccacagcgcctgcctgcccattctcagcagccatcatcagtgctgttttccctgaattatctactgcgttcactggagcactgtgtctcagaagaagctgcaagcactccacatgatcagcaaatgctgccgcatgaaggggtgtcctgcctttgtcatctctacaactgacgatactggaatctatggccccaagcagcaatgatgcacaattcccatgatcattgattattgcacagtgcagtggagtaaagggattaccgataaatttgcgaaaacatttttgctccaaaagtacctctatacagttttcattaccattgtaacaagcccagtgcagcggcgtgtagccttggttatctttgaaacaacagtcctcctcagaaagagccatttggagcagctcgctcagccacgtggcgtggccacgagcagctgcatagtgcaagggcgtcctccctctggaatctttacagagaattgacacttcttgttccagcagcatttgcacacattcctcgtgtcctgtcataatccctctgtgtaaagctgtgcatcctaggatgtcaacagtgtctacgttggcttccttttcaagtaacaatgaaacagcgtcaatatgtccatatgctactgcaagcatcagtggtgtttgtcctttggcatctttcacatcgaccgcctccgggttgtctgcaatttctagcaacagccgtaaacacagtgtgtgaccattaattactgaggcatgaagtggggttcttttggttacattgtctttcacaaagatggatgcgccctgattgataagcgcttccacacattctgtgtgtcctttaaaggcagccagatccagagcagtgcggcctttctcatccctgatgtccaggtccaccaacgactgcagaaggacttccaaggcttgatggtgcccattgtaggcagctaagtggagtggactcttagtagcaccagaatctgattcttcaaatccactgtttgttctttccaaaagcaattccagacactgcctgtgcccataggcggcagcataatgtatgctattgtaaccttccttgtcccggatagatggatttgcatcattttgaagcagaaactctagacatagtgtggcttccttttccttcagctccctggctctttcaagttcttctgaattatcatgggcatttcctaagatagtcttatttctatccatgtctgatgcagcggcgtaatgcaaagctgtgcgtccccagtcatctgtttcattaacgttggcccctgtggtcactaatgtctcaatacagtggaaatgacaattcgcagctgcatagtgcaaaggggtcctcccacacttgtcctttttatggaaatctgctccgctgctctgcaagagttttatacattccacattacctcctgcagcagcagcatgaaggcacgttcttccaaatttatctggggtgtctatttcaaagcccgatgataacaactttctgcagcagtcagagtgagcatttagggcagctaaatgtaaagggaacatgctatggattccacacttggctgtgtcagctccgctggttattaaggtgttaatcaaaagctcatgaccgtatcttgcagccacatggagaggagtgttgccgtccttatccacacagtcaatttcacctccattctgaatgagggtctgtgaccgtgtgaaccttccatggacagctgtcatgtgcagtggacttttgccatctttactctgaatgttaacatctgccccgttgtttactaacaattcaagacacaaagcaccatgagtggaggcagcagcaaaatgcaaaggggtgaacccattattgtttggctggttcacgttagcaccgtagtcaatcaactcgttaaccacagcatcctgtccattgtagcaggcgatgtgaagcgctgtatttccatagacattgatttcatcaatctccacccccaggttcaggagatgcttgacaacattaatctgtccattggaggctgcagcatgcagaggggtataacccttcttatccttacaggtcacttctgcgccatggttaatgagcaatgctacaacatccaagtggcccatgtatgctgcccagtgcagagcacgccggtccttcttgtcaaatgcattgatatttgcccctttggccaagagtaaattgaccatctccacgtggccgttcagagccgcatggtgcaaggctgtgcgcccccctcggtcggagacattgacactgctcagcaggggaatgatcacttctgcacatttgacagccttgttggctgctgccacatgaagaggggtctgccagttcttgtcccttgcattgacatcagctgagtgcttaatcaaaacctgtactgcttcttcacttctggaagcaacagcccggtgcagtggagtcagccacatgttgtccttggcatttacacgagctcctgacaaaatcaggagttcaatgatctctgcatctcccagaaatgcggccacatgaagaggggttcgtttctcagaatccagagtattcacatcttcagttttatggatgagcatccggatctcctctggatcaccgctgaagattgcctgaaccaatggtggctggtcggtgagtttgagcactgccattcttccgctccttcgcgcgcacacacatgcaggtccccggcccgcagatgtcacgccgggagccggggaagcggaagggattgccaggagaagggaaaaaatctggctcccgaatttgacagccctccccctgctcctcctccgccgccgcctcctcccgccgagaggctgacact

SEQ ID NO: 16360 - RNA, 4764 nt, Homo sapiens
  source 1..4764: mol_type = other RNA
gtagattctccttctatgagtaagagagtgggaaaagtcaaaacgcagctccatggagataacgtctcatggtgagtcactgctttgctgaaatgattcttgtactctctgctacacgacaggaaaaatgttaacgctgctttgccattaaagcaagcatttcatttcctgcttgaaatgccaactgagcaagatttccattcacttctagaaaaagacaccgcagcatattgtgcttcttcaacactgaacctctcttaattttcagtgttttggtaaagataaggtcattattgctcattagcaatttatctgctttttaaaaattcatcttctctaaacaaacgaaaaggacagaaggtgggaagcacaacaccaagaattcaaaaaaacaatggtggtggtgtggaaaattttcagtgaaatcaataccagttcaataaatcctttgaacaagttctcatttgtgaagaacccaacaggagttttaattaaatccaggatattaagagtaagattaaagttttatagctagatgaaaaatataatacagttatctgtctttgatccagatatgatagaacattatttttgaaatatctcacatacactataaaatagcaatttccagggtggaaatggaactcattataaaacgtcagagagtactgctctaattcgacacatttcttttctgtctcttcctcaagtagaaaatagcacttgagctggtgatttttatttctccttttggcacatgtgcccacacactgccatcatttctcatcaggttactgagactatgtgagcttttcagtgtacttagggtaatttctagatatttctttgtgctgcctttgtgtatatgatccactacacatctgagttttcatctcgcagaagggcatccagactgcaatgtcttctaagctctaagctggctacagactgtggctgagcagtagaagatgcgtagccctctctaaccaacgcggaagaacctgagggtcatctggaaaccttagcagtggaaatgctaggtttggcccttgggcttttggctagcccagggtcaagtgttttttttttcactttttttttgttattctaaataagatacatagcaattaaaatagagaacaaataatggatgtttcctcaccatttgtttcatttcaaataaatataaacacatttacagcaaaagtatatggacattttctctagtttggcaaaaaaaaaaaaaaaggtcagcacatcatcagttacaaatgttaagtggtcaactagaaatctgtgtcctaagaaatataaaatacaacaaagactggtacacagaaagattacatttaactccataaaaaagctacttcagttctcacttgcattttgaaggaaaaaaatgtgtatcttccattttagactgaagcattttggtcctcatgtgtagctggctgatgaactacacacacacacacatatatatatatatacacacgcacacatatatgtgtgcatgtgtatgtgcataatttttaaagagtctcattcttctttttgtacagcggttccaggtgtggaacggggtccatttgacctagaagcattttcatctacagcaagtacacaggcccctttggccagcaactcctcaactaccacctttaagccattgcgcgcagcgacgtggaggggtgtctgcagtgcattatttttttcattaataaggctctcgtcttgtatcttgtcaagtattaacaaggcacatttttcatgacctttactacaagccaaatgtaagggtgtattcaagtccttatcctttacagtcagatcagcctgggcactgttcaccaaaatatccacagcgcctgcctgcccattctcagcagccatcatcagtgctgttttccctgaattatctactgcgttcactggagcactgtgtctcagaagaagctgcaagcactccacatgatcagcaaatgctgccgcatgaaggggtgtcctgcctttgtcatctctacaactgacgatactggaatctatggccccaagcagcaatgatgcacaattcccatgatcattgattattgcacagtgcagtggagtaaagggattaccgataaatttgcgaaaacatttttgctccaaaagtacctctatacagttttcattaccattgtaacaagcccagtgcagcggcgtgtagccttggttatctttgaaacaacagtcctcctcagaaagagccatttggagcagctcgctcagccacgtggcgtggccacgagcagctgcatagtgcaagggcgtcctccctctggaatctttacagagaattgacacttcttgttccagcagcatttgcacacattcctcgtgtcctgtcataatccctctgtgtaaagctgtgcatcctaggatgtcaacagtgtctacgttggcttccttttcaagtaacaatgaaacagcgtcaatatgtccatatgctactgcaagcatcagtggtgtttgtcctttggcatctttcacatcgaccgcctccgggttgtctgcaatttctagcaacagccgtaaacacagtgtgtgaccattaattactgaggcatgaagtggggttcttttggttacattgtctttcacaaagatggatgcgccctgattgataagcgcttccacacattctgtgtgtcctttaaaggcagccagatccagagcagtgcggcctttctcatccctgatgtccaggtccaccaacgactgcagaaggacttccaaggcttgatggtgcccattgtaggcagctaagtggagtggactcttagtagcaccagaatctgattcttcaaatccactgtttgttctttccaaaagcaattccagacactgcctgtgcccataggcggcagcataatgtatgctattgtaaccttccttgtcccggatagatggatttgcatcattttgaagcagaaactctagacatagtgtggcttccttttccttcagctccctggctctttcaagttcttctgaattatcatgggcatttcctaagatagtcttatttctatccatgtctgatgcagcggcgtaatgcaaagctgtgcgtccccagtcatctgtttcattaacgttggcccctgtggtcactaatgtctcaatacagtggaaatgacaattcgcagctgcatagtgcaaaggggtcctcccacacttgtcctttttatggaaatctgctccgctgctctgcaagagttttatacattccacattacctcctgcagcagcagcatgaaggcacgttcttccaaatttatctggggtgtctatttcaaagcctgcagacagcacgtgctcattactaaacaaggatactatgctatacttttgtcccgatgataacaactttctgcagcagtcagagtgagcatttagggcagctaaatgtaaagggaacatgctatggattccacacttggctgtgtcagctccgctggttattaaggtgttaatcaaaagctcatgaccgtatcttgcagccacatggagaggagtgttgccgtccttatccacacagtcaatttcacctccattctgaatgagggtctgtgaccgtgtgaaccttccatggacagctgtcatgtgcagtggacttttgccatctttactctgaatgttaacatctgccccgttgtttactaacaattcaagacacaaagcaccatgagtggaggcagcagcaaaatgcaaaggggtgaacccattattgtttggctggttcacgttagcaccgtagtcaatcaactcgttaaccacagcatcctgtccattgtagcaggcgatgtgaagcgctgtatttccatagacattgatttcatcaatctccacccccaggttcaggagatgcttgacaacattaatctgtccattggaggctgcagcatgcagaggggtataacccttcttatccttacaggtcacttctgcgccatggttaatgagcaatgctacaacatccaagtggcccatgtatgctgcccagtgcagagcacgccggtccttcttgtcaaatgcattgatatttgcccctttggccaagagtaaattgaccatctccacgtggccgttcagagccgcatggtgcaaggctgtgcgcccccctcggtcggagacattgacactgctcagcaggggaatgatcacttctgcacatttgacagccttgttggctgctgccacatgaagaggggtctgccagttcttgtcccttgcattgacatcagctgagtgcttaatcaaaacctgtactgcttcttcacttctggaagcaacagcccggtgcagtggagtcagccacatgttgtccttggcatttacacgagctcctgacaaaatcaggagttcaatgatctctgcatctcccagaaatgcggccacatgaagaggggttcgtttctcagaatccagagtattcacatcttcagttttatggatgagcatccggatctcctctggatcaccgctgaagattgcctgaaccaatggtggctggtcggtgagtttgagcactgccattcttccgctccttcgcgcgcacacacatgcaggtccccggcccgcagatgtcacgccgggagccggggaagcggaagggattgccaggagaagggaaaaaatctggctcccgaatttgacagccctccccctgctcctcctccgccgccgcctcctcccgccgagaggctgacactggctagt

SEQ ID NO: 16361 - RNA, 5981 nt, Homo sapiens
  source 1..5981: mol_type = other RNA
gtagattctccttctatgagtaagagagtgggaaaagtcaaaacgcagctccatggagataacgtctcatggtgagtcactgctttgctgaaatgattcttgtactctctgctacacgacaggaaaaatgttaacgctgctttgccattaaagcaagcatttcatttcctgcttgaaatgccaactgagcaagatttccattcacttctagaaaaagacaccgcagcatattgtgcttcttcaacactgaacctctcttaattttcagtgttttggtaaagataaggtcattattgctcattagcaatttatctgctttttaaaaattcatcttctctaaacaaacgaaaaggacagaaggtgggaagcacaacaccaagaattcaaaaaaacaatggtggtggtgtggaaaattttcagtgaaatcaataccagttcaataaatcctttgaacaagttctcatttgtgaagaacccaacaggagttttaattaaatccaggatattaagagtaagattaaagttttatagctagatgaaaaatataatacagttatctgtctttgatccagatatgatagaacattatttttgaaatatctcacatacactataaaatagcaatttccagggtggaaatggaactcattataaaacgtcagagagtactgctctaattcgacacatttcttttctgtctcttcctcaagtagaaaatagcacttgagctggtgatttttatttctccttttggcacatgtgcccacacactgccatcatttctcatcaggttactgagactatgtgagcttttcagtgtacttagggtaatttctagatatttctttgtgctgcctttgtgtatatgatccactacacatctgagttttcatctcgcagaagggcatccagactgcaatgtcttctaagctctaagctggctacagactgtggctgagcagtagaagatgcgtagccctctctaaccaacgcggaagaacctgagggtcatctggaaaccttagcagtggaaatgctaggtttggcccttgggcttttggctagcccagggtcaagtgttttttttttcactttttttttgttattctaaataagatacatagcaattaaaatagagaacaaataatggatgtttcctcaccatttgtttcatttcaaataaatataaacacatttacagcaaaagtatatggacattttctctagtttggcaaaaaaaaaaaaaaaggtcagcacatcatcagttacaaatgttaagtggtcaactagaaatctgtgtcctaagaaatataaaatacaacaaagactggtacacagaaagattacatttaactccataaaaaagctacttcagttctcacttgcattttgaaggaaaaaaatgtgtatcttccattttagactgaagcattttggtcctcatgtgtagctggctgatgaactacacacacacacacatatatatatatatacacacgcacacatatatgtgtgcatgtgtatgtgcataatttttaaagagtctcattcttctttttgtacagcggttccaggtgtggaacggggtccatttgacctagaagctttggcagagggagcagacacagtattcactatgttgatttcatcatcaagcaactggcaatcggttttacatgctaaatcacccatttctactttctgctttcactttttttgttcctttttgcagtcacacttttcactgacttggtatgaccttgactgagaagctcattttactactgatgaacaatgctgatgattctgatgttttttaaaagttagtattttgatttaagaataaattaacaaagggtagtttcatactatttttgcatattgtgtcaaagttttggtgcaatataattttcacctgaaatgttattagataaatttgggttcaatcacttaagtgaaaattagtcacaggcttgttatagggaacactgtgttaaacaaaaaaagcaagttcaatttttcaattcatctggcaactttaacagagatcctcagaaagaagttctggatattcaaatgcttactatagagaggatataaatagttggactctctaaaaagattattacaggcattatttctgaagatggacacctttacctttggcttctagtgaggaagtaaacatcaaagtgagaagaagtttgaggcatttcctatctgcctcttcccttccctcccaggggacatgaatgtcacactgatatacttctgagaactcactgctaaatacatgaaaagaaaaattattcatagcgaacagctgcctctctgctgcattatccccaaagaacaggaattaaatacatcttttattctttatttaaaatgagaggtagactttcacagaagtatcttagatttaaagaaaatgtgaaacaaaacaaaactggggccatctgtgtgactgttccacccaacagcctcactgccctccctcgattaattccttctctactagcttctggaagcccaggccccaaataatacttgaatacaacataaacctggaattcaagcttctttcctttcctccaacacaggtgatcaaagaaaagcttctacagtccaaagtcaaaacgtttccgaatcagaatcattttcattgtacccatcctccgagcctacgttgttactgcacaggctaaccatgctacccagattggagagggtcgtcctgctcaaattgtctttttttaaacaaacgaagttgacagccatcattgtactggaaggagaaaaaggcatcatggtagccaaaatgagggccaggcagtcagccacgtctttgttaggagcgcaagccagggccggggtatgaccattttcatctacagcaagtacacaggcccctttggccagcaactcctcaactaccacctttaagccattgcgcgcagcgacgtggaggggtgtctgcagtgcattatttttttcattaataaggctctcgtcttgtatcttgtcaagtattaacaaggcacatttttcatgacctttactacaagccaaatgtaagggtgtattcaagtccttatcctttacagtcagatcagcctgggcactgttcaccaaaatatccacagcgcctgcctgcccattctcagcagccatcatcagtgctgttttccctgaattatctactgcgttcactggagcactgtgtctcagaagaagctgcaagcactccacatgatcagcaaatgctgccgcatgaaggggtgtcctgcctttgtcatctctacaactgacgatactggaatctatggccccaagcagcaatgatgcacaattcccatgatcattgattattgcacagtgcagtggagtaaagggattaccgataaatttgcgaaaacatttttgctccaaaagtacctctatacagttttcattaccattgtaacaagcccagtgcagcggcgtgtagccttggttatctttgaaacaacagtcctcctcagaaagagccatttggagcagctcgctcagccacgtggcgtggccacgagcagctgcatagtgcaagggcgtcctccctctggaatctttacagagaattgacacttcttgttccagcagcatttgcacacattcctcgtgtcctgtcataatccctctgtgtaaagctgtgcatcctaggatgtcaacagtgtctacgttggcttccttttcaagtaacaatgaaacagcgtcaatatgtccatatgctactgcaagcatcagtggtgtttgtcctttggcatctttcacatcgaccgcctccgggttgtctgcaatttctagcaacagccgtaaacacagtgtgtgaccattaattactgaggcatgaagtggggttcttttggttacattgtctttcacaaagatggatgcgccctgattgataagcgcttccacacattctgtgtgtcctttaaaggcagccagatccagagcagtgcggcctttctcatccctgatgtccaggtccaccaacgactgcagaaggacttccaaggcttgatggtgcccattgtaggcagctaagtggagtggactcttagtagcaccagaatctgattcttcaaatccactgtttgttctttccaaaagcaattccagacactgcctgtgcccataggcggcagcataatgtatgctattgtaaccttccttgtcccggatagatggatttgcatcattttgaagcagaaactctagacatagtgtggcttccttttccttcagctccctggctctttcaagttcttctgaattatcatgggcatttcctaagatagtcttatttctatccatgtctgatgcagcggcgtaatgcaaagctgtgcgtccccagtcatctgtttcattaacgttggcccctgtggtcactaatgtctcaatacagtggaaatgacaattcgcagctgcatagtgcaaaggggtcctcccacacttgtcctttttatggaaatctgctccgctgctctgcaagagttttatacattccacattacctcctgcagcagcagcatgaaggcacgttcttccaaatttatctggggtgtctatttcaaagcccgatgataacaactttctgcagcagtcagagtgagcatttagggcagctaaatgtaaagggaacatgctatggattccacacttggctgtgtcagctccgctggttattaaggtgttaatcaaaagctcatgaccgtatcttgcagccacatggagaggagtgttgccgtccttatccacacagtcaatttcacctccattctgaatgagggtctgtgaccgtgtgaaccttccatggacagctgtcatgtgcagtggacttttgccatctttactctgaatgttaacatctgccccgttgtttactaacaattcaagacacaaagcaccatgagtggaggcagcagcaaaatgcaaaggggtgaacccattattgtttggctggttcacgttagcaccgtagtcaatcaactcgttaaccacagcatcctgtccattgtagcaggcgatgtgaagcgctgtatttccatagacattgatttcatcaatctccacccccaggttcaggagatgcttgacaacattaatctgtccattggaggctgcagcatgcagaggggtataacccttcttatccttacaggtcacttctgcgccatggttaatgagcaatgctacaacatccaagtggcccatgtatgctgcccagtgcagagcacgccggtccttcttgtcaaatgcattgatatttgcccctttggccaagagtaaattgaccatctccacgtggccgttcagagccgcatggtgcaaggctgtgcgcccccctcggtcggagacattgacactgctcagcaggggaatgatcacttctgcacatttgacagccttgttggctgctgccacatgaagaggggtctgccagttcttgtcccttgcattgacatcagctgagtgcttaatcaaaacctgtactgcttcttcacttctggaagcaacagcccggtgcagtggagtcagccacatgttgtccttggcatttacacgagctcctgacaaaatcaggagttcaatgatctctgcatctcccagaaatgcggccacatgaagaggggttcgtttctcagaatccagagtattcacatcttcagttttatggatgagcatccggatctcctctggatcaccgctgaagattgcctgaaccaatggtggctggtcggtgagtttgagcactgccattcttccgctccttcgcgcgcacacacatgcaggtccccggcccgcagatgtcacgccgggagccggggaagcggaagggattgccaggagaagggaaaaaatctggctcccgaatttgacagccctccccctgctcctcctccgccgccgcctcctcccgccgagaggctgacact

SEQ ID NO: 16362 - RNA, 5961 nt, Homo sapiens
  source 1..5961: mol_type = other RNA
gtagattctccttctatgagtaagagagtgggaaaagtcaaaacgcagctccatggagataacgtctcatggtgagtcactgctttgctgaaatgattcttgtactctctgctacacgacaggaaaaatgttaacgctgctttgccattaaagcaagcatttcatttcctgcttgaaatgccaactgagcaagatttccattcacttctagaaaaagacaccgcagcatattgtgcttcttcaacactgaacctctcttaattttcagtgttttggtaaagataaggtcattattgctcattagcaatttatctgctttttaaaaattcatcttctctaaacaaacgaaaaggacagaaggtgggaagcacaacaccaagaattcaaaaaaacaatggtggtggtgtggaaaattttcagtgaaatcaataccagttcaataaatcctttgaacaagttctcatttgtgaagaacccaacaggagttttaattaaatccaggatattaagagtaagattaaagttttatagctagatgaaaaatataatacagttatctgtctttgatccagatatgatagaacattatttttgaaatatctcacatacactataaaatagcaatttccagggtggaaatggaactcattataaaacgtcagagagtactgctctaattcgacacatttcttttctgtctcttcctcaagtagaaaatagcacttgagctggtgatttttatttctccttttggcacatgtgcccacacactgccatcatttctcatcaggttactgagactatgtgagcttttcagtgtacttagggtaatttctagatatttctttgtgctgcctttgtgtatatgatccactacacatctgagttttcatctcgcagaagggcatccagactgcaatgtcttctaagctctaagctggctacagactgtggctgagcagtagaagatgcgtagccctctctaaccaacgcggaagaacctgagggtcatctggaaaccttagcagtggaaatgctaggtttggcccttgggcttttggctagcccagggtcaagtgttttttttttcactttttttttgttattctaaataagatacatagcaattaaaatagagaacaaataatggatgtttcctcaccatttgtttcatttcaaataaatataaacacatttacagcaaaagtatatggacattttctctagtttggcaaaaaaaaaaaaaaaggtcagcacatcatcagttacaaatgttaagtggtcaactagaaatctgtgtcctaagaaatataaaatacaacaaagactggtacacagaaagattacatttaactccataaaaaagctacttcagttctcacttgcattttgaaggaaaaaaatgtgtatcttccattttagactgaagcattttggtcctcatgtgtagctggctgatgaactacacacacacacacatatatatatatatacacacgcacacatatatgtgtgcatgtgtatgtgcataatttttaaagagtctcattcttctttttgtacagcggttccaggtgtggaacggggtccatttgacctagaagctttggcagagggagcagacacagtattcactatgttgatttcatcatcaagcaactggcaatcggttttacatgctaaatcacccatttctactttctgctttcactttttttgttcctttttgcagtcacacttttcactgacttggtatgaccttgactgagaagctcattttactactgatgaacaatgctgatgattctgatgttttttaaaagttagtattttgatttaagaataaattaacaaagggtagtttcatactatttttgcatattgtgtcaaagttttggtgcaatataattttcacctgaaatgttattagataaatttgggttcaatcacttaagtgaaaattagtcacaggcttgttatagggaacactgtgttaaacaaaaaaagcaagttcaatttttcaattcatctggcaactttaacagagatcctcagaaagaagttctggatattcaaatgcttactatagagaggatataaatagttggactctctaaaaagattattacaggcattatttctgaagatggacacctttacctttggcttctagtgaggaagtaaacatcaaagtgagaagaagtttgaggcatttcctatctgcctcttcccttccctcccaggggacatgaatgtcacactgatatacttctgagaactcactgctaaatacatgaaaagaaaaattattcatagcgaacagctgcctctctgctgcattatccccaaagaacaggaattaaatacatcttttattctttatttaaaatgagaggtagactttcacagaagtatcttagatttaaagaaaatgtgaaacaaaacaaaactggggccatctgtgtgactgttccacccaacagcctcactgccctccctcgattaattccttctctactagcttctggaagcccaggccccaaataatacttgaatacaacataaacctggaattcaagcttctttcctttcctccaacacaggtgatcaaagaaaagcttctacagtccaaagtcaaaacgtttccgaatcagaatcattttcattgtacccatcctccgagcctacgttgttactgcacaggctaaccatgctacccagattggagagggtcgtcctgctcaaattgtctttttttaaacaaacgaagttgacagccatcattgtactggaaggagaaaaaggcatcatggtagccaaaatgagggccaggcagtcagccacgtctttgttaggagcgcaagccagggccggggtatgaccattttcatctacagcaagtacacaggcccctttggccagcaactcctcaactaccacctttaagccattgcgcgcagcgacgtggaggggtgtctgcagtgcattatttttttcattaataaggctctcgtcttgtatcttgtcaagtattaacaaggcacatttttcatgacctttactacaagccaaatgtaagggtgtattcaagtccttatcctttacagtcagatcagcctgggcactgttcaccaaaatatccacagcgcctgcctgcccattctcagcagccatcatcagtgctgttttccctgaattatctactgcgttcactggagcactgtgtctcagaagaagctgcaagcactccacatgatcagcaaatgctgccgcatgaaggggtgtcctgcctttgtcatctctacaactgacgatactggaatctatggccccaagcagcaatgatgcacaattcccatgatcattgattattgcacagtgcagtggagtaaagggattaccgataaatttgcgaaaacatttttgctccaaaagtacctctatacagttttcattaccattgtaacaagcccagtgcagcggcgtgtagccttggttatctttgaaacaacagtcctcctcagaaagagccatttggagcagctcgctcagccacgtggcgtggccacgagcagctgcatagtgcaagggcgtcctccctctggaatctttacagagaattgacacttcttgttccagcagcatttgcacacattcctcgtgtcctgtcataatccctctgtgtaaagctgtgcatcctaggatgtcaacagtgtctacgttggcttccttttcaagtaacaatgaaacagcgtcaatatgtccatatgctactgcaagcatcagtggtgtttgtcctttggcatctttcacatcgaccgcctccgggttgtctgcaatttctagcaacagccgtaaacacagtgtgtgaccattaattactgaggcatgaagtggggttcttttggttacattgtctttcacaaagatggatgcgccctgattgataagcgcttccacacattctgtgtgtcctttaaaggcagccagatccagagcagtgcggcctttctcatccctgatgtccaggtccaccaacgactgcagaaggacttccaaggcttgatggtgcccattgtaggcagctaagtggagtggactcttagtagcaccagaatctgattcttcaaatccactgtttgttctttccaaaagcaattccagacactgcctgtgcccataggcggcagcataatgtatgctattgtaaccttccttgtcccggatagatggatttgcatcattttgaagcagaaactctagacatagtgtggcttccttttccttcagctccctggctctttcaagttcttctgaattatcatgggcatttcctaagatagtcttatttctatccatgtctgatgcagcggcgtaatgcaaagctgtgcgtccccagtcatctgtttcattaacgttggcccctgtggtcactaatgtctcaatacagtggaaatgacaattcgcagctgcatagtgcaaaggggtcctcccacacttgtcctttttatggaaatctgctccgctgctctgcaagagttttatacattccacattacctcctgcagcagcagcatgaaggcacgttcttccaaatttatctggggtgtctatttcaaagcctgcagacagcacgtgctcattactaaacaaggatactatgctatacttttgtcccgatgataacaactttctgcagcagtcagagtgagcatttagggcagctaaatgtaaagggaacatgctatggattccacacttggctgtgtcagctccgctggttattaaggtgttaatcaaaagctcatgaccgtatcttgcagccacatggagaggagtgttgccgtccttatccacacagtcaatttcacctccattctgaatgagggtctgtgaccgtgtgaaccttccatggacagctgtcatgtgcagtggacttttgccatctttactctgaatgttaacatctgccccgttgtttactaacaattcaagacacaaagcaccatgagtggaggcagcagcaaaatgcaaaggggtgaacccattattgtttggctggttcacgttagcaccgtagtcaatcaactcgttaaccacagcatcctgtccattgtagcaggcgatgtgaagcgctgtatttccatagacattgatttcatcaatctccacccccaggttcaggagatgcttgacaacattaatctgtccattggaggctgcagcatgcagaggggtataacccttcttatccttacaggtcacttctgcgccatggttaatgagcaatgctacaacatccaagtggcccatgtatgctgcccagtgcagagcacgccggtccttcttgtcaaatgcattgatatttgcccctttggccaagagtaaattgaccatctccacgtggccgttcagagccgcatggtgcaaggctgtgcgcccccctcggtcggagacattgacactgctcagcaggggaatgatcacttctgcacatttgacagccttgttggctgctgccacatgaagaggggtctgccagttcttgtcccttgcattgacatcagctgagtgcttaatcaaaacctgtactgcttcttcacttctggaagcaacagcccggtgcagtggagtcagccacatgttgtccttggcatttacacgagctcctgacaaaatcaggagttcaatgatctctgcatctcccagaaatgcggccacatgaagaggggttcgtttctcagaatccagagtattcacatcttcagttttatggatgagcatccggatctcctctggatcaccgctgaagattgcctgaaccaatggtggcaacttcttccacaggacacagggctcgggagcagcgccagcccgacatcggcggaggagcaccggaagttctgcagcactggctttctttgctcttccacctatgcaagctccttctctcttgtggct

SEQ ID NO: 16363 - RNA, 6035 nt, Homo sapiens
  source 1..6035: mol_type = other RNA
gtagattctccttctatgagtaagagagtgggaaaagtcaaaacgcagctccatggagataacgtctcatggtgagtcactgctttgctgaaatgattcttgtactctctgctacacgacaggaaaaatgttaacgctgctttgccattaaagcaagcatttcatttcctgcttgaaatgccaactgagcaagatttccattcacttctagaaaaagacaccgcagcatattgtgcttcttcaacactgaacctctcttaattttcagtgttttggtaaagataaggtcattattgctcattagcaatttatctgctttttaaaaattcatcttctctaaacaaacgaaaaggacagaaggtgggaagcacaacaccaagaattcaaaaaaacaatggtggtggtgtggaaaattttcagtgaaatcaataccagttcaataaatcctttgaacaagttctcatttgtgaagaacccaacaggagttttaattaaatccaggatattaagagtaagattaaagttttatagctagatgaaaaatataatacagttatctgtctttgatccagatatgatagaacattatttttgaaatatctcacatacactataaaatagcaatttccagggtggaaatggaactcattataaaacgtcagagagtactgctctaattcgacacatttcttttctgtctcttcctcaagtagaaaatagcacttgagctggtgatttttatttctccttttggcacatgtgcccacacactgccatcatttctcatcaggttactgagactatgtgagcttttcagtgtacttagggtaatttctagatatttctttgtgctgcctttgtgtatatgatccactacacatctgagttttcatctcgcagaagggcatccagactgcaatgtcttctaagctctaagctggctacagactgtggctgagcagtagaagatgcgtagccctctctaaccaacgcggaagaacctgagggtcatctggaaaccttagcagtggaaatgctaggtttggcccttgggcttttggctagcccagggtcaagtgttttttttttcactttttttttgttattctaaataagatacatagcaattaaaatagagaacaaataatggatgtttcctcaccatttgtttcatttcaaataaatataaacacatttacagcaaaagtatatggacattttctctagtttggcaaaaaaaaaaaaaaaggtcagcacatcatcagttacaaatgttaagtggtcaactagaaatctgtgtcctaagaaatataaaatacaacaaagactggtacacagaaagattacatttaactccataaaaaagctacttcagttctcacttgcattttgaaggaaaaaaatgtgtatcttccattttagactgaagcattttggtcctcatgtgtagctggctgatgaactacacacacacacacatatatatatatatacacacgcacacatatatgtgtgcatgtgtatgtgcataatttttaaagagtctcattcttctttttgtacagcggttccaggtgtggaacggggtccatttgacctagaagctttggcagagggagcagacacagtattcactatgttgatttcatcatcaagcaactggcaatcggttttacatgctaaatcacccatttctactttctgctttcactttttttgttcctttttgcagtcacacttttcactgacttggtatgaccttgactgagaagctcattttactactgatgaacaatgctgatgattctgatgttttttaaaagttagtattttgatttaagaataaattaacaaagggtagtttcatactatttttgcatattgtgtcaaagttttggtgcaatataattttcacctgaaatgttattagataaatttgggttcaatcacttaagtgaaaattagtcacaggcttgttatagggaacactgtgttaaacaaaaaaagcaagttcaatttttcaattcatctggcaactttaacagagatcctcagaaagaagttctggatattcaaatgcttactatagagaggatataaatagttggactctctaaaaagattattacaggcattatttctgaagatggacacctttacctttggcttctagtgaggaagtaaacatcaaagtgagaagaagtttgaggcatttcctatctgcctcttcccttccctcccaggggacatgaatgtcacactgatatacttctgagaactcactgctaaatacatgaaaagaaaaattattcatagcgaacagctgcctctctgctgcattatccccaaagaacaggaattaaatacatcttttattctttatttaaaatgagaggtagactttcacagaagtatcttagatttaaagaaaatgtgaaacaaaacaaaactggggccatctgtgtgactgttccacccaacagcctcactgccctccctcgattaattccttctctactagcttctggaagcccaggccccaaataatacttgaatacaacataaacctggaattcaagcttctttcctttcctccaacacaggtgatcaaagaaaagcttctacagtccaaagtcaaaacgtttccgaatcagaatcattttcattgtacccatcctccgagcctacgttgttactgcacaggctaaccatgctacccagattggagagggtcgtcctgctcaaattgtctttttttaaacaaacgaagttgacagccatcattgtactggaaggagaaaaaggcatcatggtagccaaaatgagggccaggcagtcagccacgtctttgttaggagcgcaagccagggccggggtatgaccattttcatctacagcaagtacacaggcccctttggccagcaactcctcaactaccacctttaagccattgcgcgcagcgacgtggaggggtgtctgcagtgcattatttttttcattaataaggctctcgtcttgtatcttgtcaagtattaacaaggcacatttttcatgacctttactacaagccaaatgtaagggtgtattcaagtccttatcctttacagtcagatcagcctgggcactgttcaccaaaatatccacagcgcctgcctgcccattctcagcagccatcatcagtgctgttttccctgaattatctactgcgttcactggagcactgtgtctcagaagaagctgcaagcactccacatgatcagcaaatgctgccgcatgaaggggtgtcctgcctttgtcatctctacaactgacgatactggaatctatggccccaagcagcaatgatgcacaattcccatgatcattgattattgcacagtgcagtggagtaaagggattaccgataaatttgcgaaaacatttttgctccaaaagtacctctatacagttttcattaccattgtaacaagcccagtgcagcggcgtgtagccttggttatctttgaaacaacagtcctcctcagaaagagccatttggagcagctcgctcagccacgtggcgtggccacgagcagctgcatagtgcaagggcgtcctccctctggaatctttacagagaattgacacttcttgttccagcagcatttgcacacattcctcgtgtcctgtcataatccctctgtgtaaagctgtgcatcctaggatgtcaacagtgtctacgttggcttccttttcaagtaacaatgaaacagcgtcaatatgtccatatgctactgcaagcatcagtggtgtttgtcctttggcatctttcacatcgaccgcctccgggttgtctgcaatttctagcaacagccgtaaacacagtgtgtgaccattaattactgaggcatgaagtggggttcttttggttacattgtctttcacaaagatggatgcgccctgattgataagcgcttccacacattctgtgtgtcctttaaaggcagccagatccagagcagtgcggcctttctcatccctgatgtccaggtccaccaacgactgcagaaggacttccaaggcttgatggtgcccattgtaggcagctaagtggagtggactcttagtagcaccagaatctgattcttcaaatccactgtttgttctttccaaaagcaattccagacactgcctgtgcccataggcggcagcataatgtatgctattgtaaccttccttgtcccggatagatggatttgcatcattttgaagcagaaactctagacatagtgtggcttccttttccttcagctccctggctctttcaagttcttctgaattatcatgggcatttcctaagatagtcttatttctatccatgtctgatgcagcggcgtaatgcaaagctgtgcgtccccagtcatctgtttcattaacgttggcccctgtggtcactaatgtctcaatacagtggaaatgacaattcgcagctgcatagtgcaaaggggtcctcccacacttgtcctttttatggaaatctgctccgctgctctgcaagagttttatacattccacattacctcctgcagcagcagcatgaaggcacgttcttccaaatttatctggggtgtctatttcaaagcctgcagacagcacgtgctcattactaaacaaggatactatgctatacttttgtcccgatgataacaactttctgcagcagtcagagtgagcatttagggcagctaaatgtaaagggaacatgctatggattccacacttggctgtgtcagctccgctggttattaaggtgttaatcaaaagctcatgaccgtatcttgcagccacatggagaggagtgttgccgtccttatccacacagtcaatttcacctccattctgaatgagggtctgtgaccgtgtgaaccttccatggacagctgtcatgtgcagtggacttttgccatctttactctgaatgttaacatctgccccgttgtttactaacaattcaagacacaaagcaccatgagtggaggcagcagcaaaatgcaaaggggtgaacccattattgtttggctggttcacgttagcaccgtagtcaatcaactcgttaaccacagcatcctgtccattgtagcaggcgatgtgaagcgctgtatttccatagacattgatttcatcaatctccacccccaggttcaggagatgcttgacaacattaatctgtccattggaggctgcagcatgcagaggggtataacccttcttatccttacaggtcacttctgcgccatggttaatgagcaatgctacaacatccaagtggcccatgtatgctgcccagtgcagagcacgccggtccttcttgtcaaatgcattgatatttgcccctttggccaagagtaaattgaccatctccacgtggccgttcagagccgcatggtgcaaggctgtgcgcccccctcggtcggagacattgacactgctcagcaggggaatgatcacttctgcacatttgacagccttgttggctgctgccacatgaagaggggtctgccagttcttgtcccttgcattgacatcagctgagtgcttaatcaaaacctgtactgcttcttcacttctggaagcaacagcccggtgcagtggagtcagccacatgttgtccttggcatttacacgagctcctgacaaaatcaggagttcaatgatctctgcatctcccagaaatgcggccacatgaagaggggttcgtttctcagaatccagagtattcacatcttcagttttatggatgagcatccggatctcctctggatcaccgctgaagattgcctgaaccaatggtggctggtcggtgagtttgagcactgccattcttccgctccttcgcgcgcacacacatgcaggtccccggcccgcagatgtcacgccgggagccggggaagcggaagggattgccaggagaagggaaaaaatctggctcccgaatttgacagccctccccctgctcctcctccgccgccgcctcctcccgccgagaggctgacact

SEQ ID NO: 16364 - RNA, 6211 nt, Homo sapiens
  source 1..6211: mol_type = other RNA
gtagattctccttctatgagtaagagagtgggaaaagtcaaaacgcagctccatggagataacgtctcatggtgagtcactgctttgctgaaatgattcttgtactctctgctacacgacaggaaaaatgttaacgctgctttgccattaaagcaagcatttcatttcctgcttgaaatgccaactgagcaagatttccattcacttctagaaaaagacaccgcagcatattgtgcttcttcaacactgaacctctcttaattttcagtgttttggtaaagataaggtcattattgctcattagcaatttatctgctttttaaaaattcatcttctctaaacaaacgaaaaggacagaaggtgggaagcacaacaccaagaattcaaaaaaacaatggtggtggtgtggaaaattttcagtgaaatcaataccagttcaataaatcctttgaacaagttctcatttgtgaagaacccaacaggagttttaattaaatccaggatattaagagtaagattaaagttttatagctagatgaaaaatataatacagttatctgtctttgatccagatatgatagaacattatttttgaaatatctcacatacactataaaatagcaatttccagggtggaaatggaactcattataaaacgtcagagagtactgctctaattcgacacatttcttttctgtctcttcctcaagtagaaaatagcacttgagctggtgatttttatttctccttttggcacatgtgcccacacactgccatcatttctcatcaggttactgagactatgtgagcttttcagtgtacttagggtaatttctagatatttctttgtgctgcctttgtgtatatgatccactacacatctgagttttcatctcgcagaagggcatccagactgcaatgtcttctaagctctaagctggctacagactgtggctgagcagtagaagatgcgtagccctctctaaccaacgcggaagaacctgagggtcatctggaaaccttagcagtggaaatgctaggtttggcccttgggcttttggctagcccagggtcaagtgttttttttttcactttttttttgttattctaaataagatacatagcaattaaaatagagaacaaataatggatgtttcctcaccatttgtttcatttcaaataaatataaacacatttacagcaaaagtatatggacattttctctagtttggcaaaaaaaaaaaaaaaggtcagcacatcatcagttacaaatgttaagtggtcaactagaaatctgtgtcctaagaaatataaaatacaacaaagactggtacacagaaagattacatttaactccataaaaaagctacttcagttctcacttgcattttgaaggaaaaaaatgtgtatcttccattttagactgaagcattttggtcctcatgtgtagctggctgatgaactacacacacacacacatatatatatatatacacacgcacacatatatgtgtgcatgtgtatgtgcataatttttaaagagtctcattcttctttttgtacagcggttccaggtgtggaacggggtccatttgacctagaagctttggcagagggagcagacacagtattcactatgttgatttcatcatcaagcaactggcaatcggttttacatgctaaatcacccatttctactttctgctttcactttttttgttcctttttgcagtcacacttttcactgacttggtatgaccttgactgagaagctcattttactactgatgaacaatgctgatgattctgatgttttttaaaagttagtattttgatttaagaataaattaacaaagggtagtttcatactatttttgcatattgtgtcaaagttttggtgcaatataattttcacctgaaatgttattagataaatttgggttcaatcacttaagtgaaaattagtcacaggcttgttatagggaacactgtgttaaacaaaaaaagcaagttcaatttttcaattcatctggcaactttaacagagatcctcagaaagaagttctggatattcaaatgcttactatagagaggatataaatagttggactctctaaaaagattattacaggcattatttctgaagatggacacctttacctttggcttctagtgaggaagtaaacatcaaagtgagaagaagtttgaggcatttcctatctgcctcttcccttccctcccaggggacatgaatgtcacactgatatacttctgagaactcactgctaaatacatgaaaagaaaaattattcatagcgaacagctgcctctctgctgcattatccccaaagaacaggaattaaatacatcttttattctttatttaaaatgagaggtagactttcacagaagtatcttagatttaaagaaaatgtgaaacaaaacaaaactggggccatctgtgtgactgttccacccaacagcctcactgccctccctcgattaattccttctctactagcttctggaagcccaggccccaaataatacttgaatacaacataaacctggaattcaagcttctttcctttcctccaacacaggtgatcaaagaaaagcttctacagtccaaagtcaaaacgtttccgaatcagaatcattttcattgtacccatcctccgagcctacgttgttactgcacaggctaaccatgctacccagattggagagggtcgtcctgctcaaattgtctttttttaaacaaacgaagttgacagccatcattgtactggaaggagaaaaaggcatcatggtagccaaaatgagggccaggcagtcagccacgtctttgttaggagcgcaagccagggccggggtatgacctgggcgtaaatgcagacaaggcagtggttagtcctggggagcctagaggaggcacgagcattccacagtacatctcggatgatctcacaggcggagatgtatgttgagttagaaatcatgccaggtaaaacgaggagttacttctcacaagtcatgctaggggtgaggcattttcatctacagcaagtacacaggcccctttggccagcaactcctcaactaccacctttaagccattgcgcgcagcgacgtggaggggtgtctgcagtgcattatttttttcattaataaggctctcgtcttgtatcttgtcaagtattaacaaggcacatttttcatgacctttactacaagccaaatgtaagggtgtattcaagtccttatcctttacagtcagatcagcctgggcactgttcaccaaaatatccacagcgcctgcctgcccattctcagcagccatcatcagtgctgttttccctgaattatctactgcgttcactggagcactgtgtctcagaagaagctgcaagcactccacatgatcagcaaatgctgccgcatgaaggggtgtcctgcctttgtcatctctacaactgacgatactggaatctatggccccaagcagcaatgatgcacaattcccatgatcattgattattgcacagtgcagtggagtaaagggattaccgataaatttgcgaaaacatttttgctccaaaagtacctctatacagttttcattaccattgtaacaagcccagtgcagcggcgtgtagccttggttatctttgaaacaacagtcctcctcagaaagagccatttggagcagctcgctcagccacgtggcgtggccacgagcagctgcatagtgcaagggcgtcctccctctggaatctttacagagaattgacacttcttgttccagcagcatttgcacacattcctcgtgtcctgtcataatccctctgtgtaaagctgtgcatcctaggatgtcaacagtgtctacgttggcttccttttcaagtaacaatgaaacagcgtcaatatgtccatatgctactgcaagcatcagtggtgtttgtcctttggcatctttcacatcgaccgcctccgggttgtctgcaatttctagcaacagccgtaaacacagtgtgtgaccattaattactgaggcatgaagtggggttcttttggttacattgtctttcacaaagatggatgcgccctgattgataagcgcttccacacattctgtgtgtcctttaaaggcagccagatccagagcagtgcggcctttctcatccctgatgtccaggtccaccaacgactgcagaaggacttccaaggcttgatggtgcccattgtaggcagctaagtggagtggactcttagtagcaccagaatctgattcttcaaatccactgtttgttctttccaaaagcaattccagacactgcctgtgcccataggcggcagcataatgtatgctattgtaaccttccttgtcccggatagatggatttgcatcattttgaagcagaaactctagacatagtgtggcttccttttccttcagctccctggctctttcaagttcttctgaattatcatgggcatttcctaagatagtcttatttctatccatgtctgatgcagcggcgtaatgcaaagctgtgcgtccccagtcatctgtttcattaacgttggcccctgtggtcactaatgtctcaatacagtggaaatgacaattcgcagctgcatagtgcaaaggggtcctcccacacttgtcctttttatggaaatctgctccgctgctctgcaagagttttatacattccacattacctcctgcagcagcagcatgaaggcacgttcttccaaatttatctggggtgtctatttcaaagcctgcagacagcacgtgctcattactaaacaaggatactatgctatacttttgtcccgatgataacaactttctgcagcagtcagagtgagcatttagggcagctaaatgtaaagggaacatgctatggattccacacttggctgtgtcagctccgctggttattaaggtgttaatcaaaagctcatgaccgtatcttgcagccacatggagaggagtgttgccgtccttatccacacagtcaatttcacctccattctgaatgagggtctgtgaccgtgtgaaccttccatggacagctgtcatgtgcagtggacttttgccatctttactctgaatgttaacatctgccccgttgtttactaacaattcaagacacaaagcaccatgagtggaggcagcagcaaaatgcaaaggggtgaacccattattgtttggctggttcacgttagcaccgtagtcaatcaactcgttaaccacagcatcctgtccattgtagcaggcgatgtgaagcgctgtatttccatagacattgatttcatcaatctccacccccaggttcaggagatgcttgacaacattaatctgtccattggaggctgcagcatgcagaggggtataacccttcttatccttacaggtcacttctgcgccatggttaatgagcaatgctacaacatccaagtggcccatgtatgctgcccagtgcagagcacgccggtccttcttgtcaaatgcattgatatttgcccctttggccaagagtaaattgaccatctccacgtggccgttcagagccgcatggtgcaaggctgtgcgcccccctcggtcggagacattgacactgctcagcaggggaatgatcacttctgcacatttgacagccttgttggctgctgccacatgaagaggggtctgccagttcttgtcccttgcattgacatcagctgagtgcttaatcaaaacctgtactgcttcttcacttctggaagcaacagcccggtgcagtggagtcagccacatgttgtccttggcatttacacgagctcctgacaaaatcaggagttcaatgatctctgcatctcccagaaatgcggccacatgaagaggggttcgtttctcagaatccagagtattcacatcttcagttttatggatgagcatccggatctcctctggatcaccgctgaagattgcctgaaccaatggtggctggtcggtgagtttgagcactgccattcttccgctccttcgcgcgcacacacatgcaggtccccggcccgcagatgtcacgccgggagccggggaagcggaagggattgccaggagaagggaaaaaatctggctcccgaatttgacagccctccccctgctcctcctccgccgccgcctcctcccgccgagaggctgacactggctagt

SEQ ID NO: 16365 - RNA, 7923 nt, Homo sapiens
  source 1..7923: mol_type = other RNA
gtagattctccttctatgagtaagagagtgggaaaagtcaaaacgcagctccatggagataacgtctcatggtgagtcactgctttgctgaaatgattcttgtactctctgctacacgacaggaaaaatgttaacgctgctttgccattaaagcaagcatttcatttcctgcttgaaatgccaactgagcaagatttccattcacttctagaaaaagacaccgcagcatattgtgcttcttcaacactgaacctctcttaattttcagtgttttggtaaagataaggtcattattgctcattagcaatttatctgctttttaaaaattcatcttctctaaacaaacgaaaaggacagaaggtgggaagcacaacaccaagaattcaaaaaaacaatggtggtggtgtggaaaattttcagtgaaatcaataccagttcaataaatcctttgaacaagttctcatttgtgaagaacccaacaggagttttaattaaatccaggatattaagagtaagattaaagttttatagctagatgaaaaatataatacagttatctgtctttgatccagatatgatagaacattatttttgaaatatctcacatacactataaaatagcaatttccagggtggaaatggaactcattataaaacgtcagagagtactgctctaattcgacacatttcttttctgtctcttcctcaagtagaaaatagcacttgagctggtgatttttatttctccttttggcacatgtgcccacacactgccatcatttctcatcaggttactgagactatgtgagcttttcagtgtacttagggtaatttctagatatttctttgtgctgcctttgtgtatatgatccactacacatctgagttttcatctcgcagaagggcatccagactgcaatgtcttctaagctctaagctggctacagactgtggctgagcagtagaagatgcgtagccctctctaaccaacgcggaagaacctgagggtcatctggaaaccttagcagtggaaatgctaggtttggcccttgggcttttggctagcccagggtcaagtgttttttttttcactttttttttgttattctaaataagatacatagcaattaaaatagagaacaaataatggatgtttcctcaccatttgtttcatttcaaataaatataaacacatttacagcaaaagtatatggacattttctctagtttggcaaaaaaaaaaaaaaaggtcagcacatcatcagttacaaatgttaagtggtcaactagaaatctgtgtcctaagaaatataaaatacaacaaagactggtacacagaaagattacatttaactccataaaaaagctacttcagttctcacttgcattttgaaggaaaaaaatgtgtatcttccattttagactgaagcattttggtcctcatgtgtagctggctgatgaactacacacacacacacatatatatatatatacacacgcacacatatatgtgtgcatgtgtatgtgcataatttttaaagagtctcattcttctttttgtacagcggttccaggtgtggaacggggtccatttgacctagaagctttggcagagggagcagacacagtattcactatgttgatttcatcatcaagcaactggcaatcggttttacatgctaaatcacccatttctactttctgctttcactttttttgttcctttttgcagtcacacttttcactgacttggtatgaccttgactgagaagctcattttactactgatgaacaatgctgatgattctgatgttttttaaaagttagtattttgatttaagaataaattaacaaagggtagtttcatactatttttgcatattgtgtcaaagttttggtgcaatataattttcacctgaaatgttattagataaatttgggttcaatcacttaagtgaaaattagtcacaggcttgttatagggaacactgtgttaaacaaaaaaagcaagttcaatttttcaattcatctggcaactttaacagagatcctcagaaagaagttctggatattcaaatgcttactatagagaggatataaatagttggactctctaaaaagattattacaggcattatttctgaagatggacacctttacctttggcttctagtgaggaagtaaacatcaaagtgagaagaagtttgaggcatttcctatctgcctcttcccttccctcccaggggacatgaatgtcacactgatatacttctgagaactcactgctaaatacatgaaaagaaaaattattcatagcgaacagctgcctctctgctgcattatccccaaagaacaggaattaaatacatcttttattctttatttaaaatgagaggtagactttcacagaagtatcttagatttaaagaaaatgtgaaacaaaacaaaactggggccatctgtgtgactgttccacccaacagcctcactgccctccctcgattaattccttctctactagcttctggaagcccaggccccaaataatacttgaatacaacataaacctggaattcaagcttctttcctttcctccaacacaggtgatcaaagaaaagcttctacagtccaaagtcaaaacgtttccgaatcagaatcattttcattgtacccatcctccgagcctacgttgttactgcacaggctaaccatgctacccagattggagagggtcgtcctgctcaaattgtctttttttaaacaaacgaagttgacagccatcattgtactggaaggagaaaaaggcatcatggtagccaaaatgagggccaggcagtcagccacgtctttgttaggagcgcaagccagggccggggtatgacctgggcgtaaatgcagacaaggcagtggttagtcctggggagcctagaggaggcacgagcattccacagtacatctcggatgatctcacaggcggagatgtatgttgagttagaaatcatgccaggtaaaacgaggagttacttctcacaagtcatgctaggggtgaggctagagggggagggagggggagacattttatggagggctttttatttttgttttcagctcatatgactatgacaagcacaatatcatccaaagttaggcaggattccagccttcatttagtgaacacaaacacaagggggtgggtgtgggacacaattccacaataaacagcaacaggacaatcaggaggatgtttccgcctgagagcacacacacaccatgagcctcaggcctgggcctgagaaggactctcattctgagaacaatgactttccattgttaggtaattgtgtgtccaattagaaaagatattgaaaattagatgactgcaaaagtgagtaatgaagttttgtcactttatatatgcttcatagaaaatagacaccaataactggttttagaaaaatggaatcatttcagtagatcagagacaggaaagcacaggttgtttgtgattaaaaatgtacaatcatttaggagaaatttaacaaattttttttttgacagagtttcactctgtcacccaggctggattgtagtggcatggggccttgattttactacagccttgtcttccgggctcaagcaatcctcccacctcagcctcccgagtagctgggactataggtgtgtgccactactaccggctgattttttctttttttggttttttttttttgagtcaaggtcttgctatgtttcccaggctgttctcaaactcctgggctcaagcgatcctcccaccttggcttcccaaagtcctgggattaaaggcgtgagccatcacacctggcctaacagaatatttaaaaatggccactcaccaatcaaagtctcaaatctaaaatgtaatggatgtgagaaaattactatgcttgtcataattagaaccatgttattctcatttagactcaatggatccaatccagataagaaaactgtcttaactcataatataggttccttggggaggtagattaagtctttgacttgattatttccttatccaacctttatcctactggcctgaaaagggttagctgccttctcagctggccaaagtttccactacacagtgagtagggcacttgctcagtaattcagaggaatggctcaatgaaacttaacgttttgttgttttgtttatcatcactcgacctgctctccccaccctgccctttaggacatcattcctttttctggtatgaaaacaaataagaatgaacaggtagtttaacattccatttcacgaaagtcagtgatgagtaaaggaattatggttgtactgctatataaaattgccccaaacgttcccaggcctttgggatgcaggtgcgcaccaacccagggctcttgttcctaaggtcactatcagctgaacaaaccttcaatgcagcagatttacaccaggaaaagcaaaactaatttattctattctctttgaccattttggagaaaaactgtgggcctctgcaggccaaccctaagtctacagtagtgttaagagggtgagggaaggtgaggcgggaaaaccaaggaaatggagtaatagggaactttctgcacttcctagatgagtcaggtgggggacacagcagggtacatgctaggatacatggggctgcaaaatcaaaactaataagagttagctaatgataatcagtatggctgcttacttctgagaaataggcatgagctgctaattccaataccattttcatctacagcaagtacacaggcccctttggccagcaactcctcaactaccacctttaagccattgcgcgcagcgacgtggaggggtgtctgcagtgcattatttttttcattaataaggctctcgtcttgtatcttgtcaagtattaacaaggcacatttttcatgacctttactacaagccaaatgtaagggtgtattcaagtccttatcctttacagtcagatcagcctgggcactgttcaccaaaatatccacagcgcctgcctgcccattctcagcagccatcatcagtgctgttttccctgaattatctactgcgttcactggagcactgtgtctcagaagaagctgcaagcactccacatgatcagcaaatgctgccgcatgaaggggtgtcctgcctttgtcatctctacaactgacgatactggaatctatggccccaagcagcaatgatgcacaattcccatgatcattgattattgcacagtgcagtggagtaaagggattaccgataaatttgcgaaaacatttttgctccaaaagtacctctatacagttttcattaccattgtaacaagcccagtgcagcggcgtgtagccttggttatctttgaaacaacagtcctcctcagaaagagccatttggagcagctcgctcagccacgtggcgtggccacgagcagctgcatagtgcaagggcgtcctccctctggaatctttacagagaattgacacttcttgttccagcagcatttgcacacattcctcgtgtcctgtcataatccctctgtgtaaagctgtgcatcctaggatgtcaacagtgtctacgttggcttccttttcaagtaacaatgaaacagcgtcaatatgtccatatgctactgcaagcatcagtggtgtttgtcctttggcatctttcacatcgaccgcctccgggttgtctgcaatttctagcaacagccgtaaacacagtgtgtgaccattaattactgaggcatgaagtggggttcttttggttacattgtctttcacaaagatggatgcgccctgattgataagcgcttccacacattctgtgtgtcctttaaaggcagccagatccagagcagtgcggcctttctcatccctgatgtccaggtccaccaacgactgcagaaggacttccaaggcttgatggtgcccattgtaggcagctaagtggagtggactcttagtagcaccagaatctgattcttcaaatccactgtttgttctttccaaaagcaattccagacactgcctgtgcccataggcggcagcataatgtatgctattgtaaccttccttgtcccggatagatggatttgcatcattttgaagcagaaactctagacatagtgtggcttccttttccttcagctccctggctctttcaagttcttctgaattatcatgggcatttcctaagatagtcttatttctatccatgtctgatgcagcggcgtaatgcaaagctgtgcgtccccagtcatctgtttcattaacgttggcccctgtggtcactaatgtctcaatacagtggaaatgacaattcgcagctgcatagtgcaaaggggtcctcccacacttgtcctttttatggaaatctgctccgctgctctgcaagagttttatacattccacattacctcctgcagcagcagcatgaaggcacgttcttccaaatttatctggggtgtctatttcaaagcctgcagacagcacgtgctcattactaaacaaggatactatgctatacttttgtcccgatgataacaactttctgcagcagtcagagtgagcatttagggcagctaaatgtaaagggaacatgctatggattccacacttggctgtgtcagctccgctggttattaaggtgttaatcaaaagctcatgaccgtatcttgcagccacatggagaggagtgttgccgtccttatccacacagtcaatttcacctccattctgaatgagggtctgtgaccgtgtgaaccttccatggacagctgtcatgtgcagtggacttttgccatctttactctgaatgttaacatctgccccgttgtttactaacaattcaagacacaaagcaccatgagtggaggcagcagcaaaatgcaaaggggtgaacccattattgtttggctggttcacgttagcaccgtagtcaatcaactcgttaaccacagcatcctgtccattgtagcaggcgatgtgaagcgctgtatttccatagacattgatttcatcaatctccacccccaggttcaggagatgcttgacaacattaatctgtccattggaggctgcagcatgcagaggggtataacccttcttatccttacaggtcacttctgcgccatggttaatgagcaatgctacaacatccaagtggcccatgtatgctgcccagtgcagagcacgccggtccttcttgtcaaatgcattgatatttgcccctttggccaagagtaaattgaccatctccacgtggccgttcagagccgcatggtgcaaggctgtgcgcccccctcggtcggagacattgacactgctcagcaggggaatgatcacttctgcacatttgacagccttgttggctgctgccacatgaagaggggtctgccagttcttgtcccttgcattgacatcagctgagtgcttaatcaaaacctgtactgcttcttcacttctggaagcaacagcccggtgcagtggagtcagccacatgttgtccttggcatttacacgagctcctgacaaaatcaggagttcaatgatctctgcatctcccagaaatgcggccacatgaagaggggttcgtttctcagaatccagagtattcacatcttcagttttatggatgagcatccggatctcctctggatcaccgctgaagattgcctgaaccaatggtggctggtcggtgagtttgagcactgccattcttccgctccttcgcgcgcacacacatgcaggtccccggcccgcagatgtcacgccgggagccggggaagcggaagggattgccaggagaagggaaaaaatctggctcccgaatttgacagccctccccctgctcctcctccgccgccgcctcctcccgccgagaggctgacactggctagt

SEQ ID NO: 16366 - RNA, 478 nt, Homo sapiens
  source 1..478: mol_type = other RNA
gtcactgatgtctgtagctgagaatggtgaaagtaatcccagttatcgcaaccaaggagctgataacattcatgcccgtgacaccttgaccaataagtgctccccagaatggatatcctgtgaggacaacaaggggaagtctttgggagaaaccgatgtaattaagtgcaaatatagttccaaagcccacaatgattagagcaagcaggatctgggtagcccccaagactcttggctctcccttcagaaaatccagcagagagctatgaggtctgtagggaaatgcagtcaatacagtttcgtttggttttatagtgatgacgtgagttgcccttctgtcctgggatgttgactccatgattctatggcagaactctagtaagggaaagagtgagcaaacattgccgcccaaatcatgatctacctctccaccagagtcacatggagccctcagagatgagcccttagtgatgactct

SEQ ID NO: 16367 - RNA, 529 nt, Homo sapiens
  source 1..529: mol_type = other RNA
gtcactgatgtctgtagctgagaatggtgaaagtaatcccagttatcgcaaccaaggagctgataacattcatgcccgtgacaccttgacccagaagttttgatttcttatcggttactgtgaggtatcctgtaagaataaaaataagtgctccccagaatggatatcctgtgaggacaacaaggggaagtctttgggagaaaccgatgtaattaagtgcaaatatagttccaaagcccacaatgattagagcaagcaggatctgggtagcccccaagactcttggctctcccttcagaaaatccagcagagagctatgaggtctgtagggaaatgcagtcaatacagtttcgtttggttttatagtgatgacgtgagttgcccttctgtcctgggatgttgactccatgattctatggcagaactctagtaagggaaagagtgagcaaacattgccgcccaaatcatgatctacctctccaccagagtcacatggagccctcagagatgagcccttagtgatgactct

SEQ ID NO: 16368 - RNA, 2926 nt, Homo sapiens
  source 1..2926: mol_type = other RNA
gtccacttctgcctgccctgccaggacggagggcatgggcctgtgtggaaaccccagggctccctgactcccatgaggcttctcagggacttcctgccccgagggtcccagcatctcccaggtggaggtcctcaaggatgcccccaccagctccccacagctactgtagcaggaagtccttcttcccgaacccagagcccagggcggatctcccgggctgcgcgccaaggtggaaaccctcagggtcctgggggaaccagggcccaggtctggactccattcgggaccttcccagctccggggaatcacaacacagaagtaccccaggggctgaagccactaggcccccgtggagccctggccacctgccagagccctggccctacgcctggaaggcagagtcctggtctccagactcgctggggctgggtgttcctgtcccccgcggagggcctgcgcaggggagagctggtcccgcgtgggcctcccgattctccccacgcggaaccagctccacaaaactctgttctccaaggctccttaggcacaagacttgagttctcactaacttacccaaaacacaaccaaacacaatccctgcctggaccctctcctagcgaagcagattggagcgctgctggctcaccctcatggggcccgagaggctcaaggaccctgggggagaagttgaagcccacacaggcgcaggacacggtgggtgggagaggcggccgggcctccagaagacggggcgcttggggctgaaggggcgtgaactcccttcaagggccccttggggcggtcgggaccatcaccagatctgctgagagactgggaggagtgagttccatctgcaggggagctcaggagactcttgaactggacttagcccgagtcctgcaggtagaaggcgccgacccccacctctgctccaagccactgcctcctgaggccacagtccaactggaagcagctccacactcggtctccccagaggccgtgtccccgtccaaggccgtcttacagcagacacagaacaggaaggaaaatttggcaaacgtgtggccccacagagtccagggagaagccagcccggccccaggccggccgcatggatgctggccccgtgcacggcagccccaggccacgcaggctcccggtcccttcctagatcatgccagccagccagggcggcaggaagaggcccaccgtccccagcaggcagacgatgatgaacatccagaggaagatgcggtcgatgaccatggccacgtacttccagtcctccttcaccgagaagtctgtgtcttcggccttcaggtggtctgcaatgtactggacgccctccaccgcccgggtcagggccggcgacaggggcaggtgcgggggcggcgctttggtgctgcgggtcttgaccgtggcgctcggggacaccgaagagggctccttcttgcatgtgcatttgcacggagagggctggtctgggggtgggagctcagccgagtgggtgttgcgagaggccagggcgccggcagcctggccatctgcctcgggggcggcatcgtctcggggaacacagtactggatgctccgagaccggcaccggacgccgccttccaccgcttcgccagggctggacatgtgctggacgctgagggacctggctttggccagccctggtgcctgggtgccgtggggcgggcggcagggtccaggcgaggggtgggggctggctttctcagcttccaggggctgctgaggagggagctggtcggagggtgacttgcaggaaggcccaggctcagccggcacatccagggggacacagaaggacggtgagggcgggtgcaggctctgggtgccgctcgtggcagggggctccccttctggctcgggccagaagcgcggggcactggccatcttatgcatggactcgatgagccgccggcaattgtccttgaccacggacggccgcttcatgaggagcaggcgtggcacgatgtccaggaagaccctgcgtacccaggtgggcatggtgtgcgtgcgtggcgagcggtggtgcacgttgagcacgaagaccgtgatgacgatggacagggtgacgaagatcatggtgaacagcaggtactcgccgatgagtgggatgaccagtgaggtggacgggatgatctcggtgatgagcagcaggaagacggtgagcgacagcagcacggagatgcacagcgtgatcttctcgccacactcggagggcaggtagaagaccagcacggtgaggcaggagatgagcaggcaggggatgatgaggttgatggtgtagaagagcggcagccgccggatgacgaaggcataggtgatgtccgggtagatctcggcacagcactcgtacttcctggtgttgtaggtgcccacggcatccacgatgacccactcgccactctcccagaagtccagctggtccacgcggctgtgcatgttcaccaggtcgatcttggccttgtcgtaggtccaggagccgaatttcatggtgcagttctgctggtcgaaggggaagaaggtgacgtcgatgctgcaggagctcttgtaaatggccgggggagtccactgcacccgcccgtcatggaacaggtgggccttggtcaggtgggtgaccgcgaagtccccgtcagcaccctctccagggcaccctgcagtccacactattctcccagaaaggccaggatggggtctgatggcgaaaagcactcctgcccaaaagggctctcctgcagttgttgtagaggacgatgtccggccgccagatgagctcggaggggatgcggatggaggtgacattctcatagtcagctgggtcccagcgcagcttgtagtcgtgccactcctgcttcacccatacgttcgtggtcatcatctggttcttctcatccta

SEQ ID NO: 16369 - RNA, 2756 nt, Homo sapiens
  source 1..2756: mol_type = other RNA
gtccacttctgcctgccctgccaggacggagggcatgggcctgtgtggaaaccccagggctccctgactcccatgaggcttctcagggacttcctgccccgagggtcccagcatctcccaggtggaggtcctcaaggatgcccccaccagctccccacagctactgtagcaggaagtccttcttcccgaacccagagcccagggcggatctcccgggctgcgcgccaaggtggaaaccctcagggtcctgggggaaccagggcccaggtctggactccattcgggaccttcccagctccggggaatcacaacacagaagtaccccaggggctgaagccactaggcccccgtggagccctggccacctgccagagccctggccctacgcctggaaggcagagtcctggtctccagactcgctggggctgggtgttcctgtcccccgcggagggcctgcgcaggggagagctggtcccgcgtgggcctcccgattctccccacgcggaaccagctccacaaaactctgttctccaaggctccttaggcacaagacttgagttctcactaacttacccaaaacacaaccaaacacaatccctgcctggaccctctcctagcgaagcagattggagcgctgctggctcaccctcatggggcccgagaggctcaaggaccctgggggagaagttgaagcccacacaggcgcaggacacggtgggtgggagaggcggccgggcctccagaagacggggcgcttggggctgaaggggcgtgaactcccttcaagggccccttggggcggtcgggaccatcaccagatctgctgagagactgggaggagtgagttccatctgcaggggagctcaggagactcttgaactggacttagcccgagtcctgcaggtagaaggcgccgacccccacctctgctccaagccactgcctcctgaggccacagtccaactggaagcagctccacactcggtctccccagaggccgtgtccccgtccaaggccgtcttacagcagacacagaacaggaaggaaaatttggcaaacgtgtggccccacagagtccagggagaagccagcccggccccaggccggccgcatggatgctggccccgtgcacggcagccccaggccacgcaggctcccggtcccttcctagatcatgccagccagccagggcggcaggaagaggcccaccgtccccagcaggcagacgatgatgaacatccagaggaagatgcggtcgatgaccatggccacgtacttccagtcctccttcaccgagaagtctgtgtcttcggccttcaggtggtctgcaatgtactggacgccctccaccgcccgggtcagggccggcgacaggggcaggtgcgggggcggcgctttggtgctgcgggtcttgaccgtggcgctcggggacaccgaagagggctccttcttgcatgtgcatttgcacggagagggctggtctgggggtgggagctcagccgagtgggtgttgcgagaggccagggcgccggcagcctggccatctgcctcgggggcggcatcgtctcggggaacacagtactggatgctccgagaccggcaccggacgccgccttccaccgcttcgccagggctggacatgtgctggacgctgagggacctggctttggccagccctggtgcctgggtgccgtggggcgggcggcagggtccaggcgaggggtgggggctggctttctcagcttccaggggctgctgaggagggagctggtcggagggtgacttgcaggaaggcccaggctcagccggcacatccagggggacacagaaggacggtgagggcgggtgcaggctctgggtgccgctcgtggcagggggctccccttctggctcgggccagaagcgcggggcactggccatcttatgcatggactcgatgagccgccggcaattgtccttgaccacggacggccgcttcatgaggagcaggcgtggcacgatgtccaggaagaccctgcgtacccaggtgggcatggtgtgcgtgcgtggcgagcggtggtgcacgttgagcacgaagaccgtgatgacgatggacagggtgacgaagatcatggtgaacagcaggtactcgccgatgagtgggatgaccagtgaggtggacgggatgatctcggtgatgagcagcaggaagacggtgagcgacagcagcacggagatgcacagcgtgatcttctcgccacactcggagggcaggtagaagaccagcacggtgaggcaggagatgagcaggcaggggatgatgaggttgatggtgtagaagagcggcagccgccggatgacgaaggcataggtgatgtccgggtagatctcggcacagcactcgtacttcctggtgttgtaggtgcccacggcatccacgatgacccactcgccactctcccagaagtccagctggtccacgcggctgtgcatgttcaccaggtcgatcttggccttgtcgtaggtccaggagccgaatttcatggtgcagttctgctggtcgaaggggaagaaggtgacgtcgatgctgcaggagctcttgtaaatggccgggggagtccactgcacccgcccgtcatggaacaggtgggccttggtcaggtgggtgaccgcgaagtccccgtcagcactggtgggggctgcagtctttggagggccgtggtcctggtgaggctgtggaagtggggggggctgcagtactcggggggctgtggtcc

SEQ ID NO: 16370 - RNA, 3235 nt, Homo sapiens
  source 1..3235: mol_type = other RNA
gtccacttctgcctgccctgccaggacggagggcatgggcctgtgtggaaaccccagggctccctgactcccatgaggcttctcagggacttcctgccccgagggtcccagcatctcccaggtggaggtcctcaaggatgcccccaccagctccccacagctactgtagcaggaagtccttcttcccgaacccagagcccagggcggatctcccgggctgcgcgccaaggtggaaaccctcagggtcctgggggaaccagggcccaggtctggactccattcgggaccttcccagctccggggaatcacaacacagaagtaccccaggggctgaagccactaggcccccgtggagccctggccacctgccagagccctggccctacgcctggaaggcagagtcctggtctccagactcgctggggctgggtgttcctgtcccccgcggagggcctgcgcaggggagagctggtcccgcgtgggcctcccgattctccccacgcggaaccagctccacaaaactctgttctccaaggctccttaggcacaagacttgagttctcactaacttacccaaaacacaaccaaacacaatccctgcctggaccctctcctagcgaagcagattggagcgctgctggctcaccctcatggggcccgagaggctcaaggaccctgggggagaagttgaagcccacacaggcgcaggacacggtgggtgggagaggcggccgggcctccagaagacggggcgcttggggctgaaggggcgtgaactcccttcaagggccccttggggcggtcgggaccatcaccagatctgctgagagactgggaggagtgagttccatctgcaggggagctcaggagactcttgaactggacttagcccgagtcctgcaggtagaaggcgccgacccccacctctgctccaagccactgcctcctgaggccacagtccaactggaagcagctccacactcggtctccccagaggccgtgtccccgtccaaggccgtcttacagcagacacagaacaggaaggaaaatttggcaaacgtgtggccccacagagtccagggagaagccagcccggccccaggccggccgcatggatgctggccccgtgcacggcagccccaggccacgcaggctcccggtcccttcctagatcatgccagccagccagggcggcaggaagaggcccaccgtccccagcaggcagacgatgatgaacatccagaggaagatgcggtcgatgaccatggccacgtacttccagtcctccttcaccgagaagtctgtgtcttcggccttcaggtggtctgcaatgtactggacgccctccaccgcccgggtcagggccggcgacaggggcaggtgcgggggcggcgctttggtgctgcgggtcttgaccgtggcgctcggggacaccgaagagggctccttcttgcatgtgcatttgcacggagagggctggtctgggggtgggagctcagccgagtgggtgttgcgagaggccagggcgccggcagcctggccatctgcctcgggggcggcatcgtctcggggaacacagtactggatgctccgagaccggcaccggacgccgccttccaccgcttcgccagggctggacatgtgctggacgctgagggacctggctttggccagccctggtgcctgggtgccgtggggcgggcggcagggtccaggcgaggggtgggggctggctttctcagcttccaggggctgctgaggagggagctggtcggagggtgacttgcaggaaggcccaggctcagccggcacatccagggggacacagaaggacggtgagggcgggtgcaggctctgggtgccgctcgtggcagggggctccccttctggctcgggccagaagcgcggggcactggccatcttatgcatggactcgatgagccgccggcaattgtccttgaccacggacggccgcttcatgaggagcaggcgtggcacgatgtccaggaagaccctgcgtacccaggtgggcatggtgtgcgtgcgtggcgagcggtggtgcacgttgagcacgaagaccgtgatgacgatggacagggtgacgaagatcatggtgaacagcaggtactcgccgatgagtgggatgaccagtgaggtggacgggatgatctcggtgatgagcagcaggaagacggtgagcgacagcagcacggagatgcacagcgtgatcttctcgccacactcggagggcaggtagaagaccagcacggtgaggcaggagatgagcaggcaggggatgatgaggttgatggtgtagaagagcggcagccgccggatgacgaaggcataggtgatgtccgggtagatctcggcacagcactcgtacttcctggtgttgtaggtgcccacggcatccacgatgacccactcgccactctcccagaagtccagctggtccacgcggctgtgcatgttcaccaggtcgatcttggccttgtcgtaggtccaggagccgaatttcatggtgcagttctgctggtcgaaggggaagaaggtgacgtcgatgctgcaggagctcttgtaaatggccgggggagtccactgcacccgcccgtcatggaacaggtgggccttggtcaggtgggtgaccgcgaagtccccgtcagcattgttgtagaggacgatgtccggccgccagatgagctcggaggggatgcggatggaggtgacattctcatagtcagctgggtcccagcgcagcttgtagtcgtgccactcctgcttcacccatacgttcgtggtcatcatctggttcttctcatccacgtcaatgagctgagcgatggacaggccgaagcggacgaggaccacgtccgagatgttggccacgggtcgggaccacttgttgtaaccggagaagagtttcttcaggagccgctcctcggcgtgggcccgggtctccacatggctgctggcgcgcaggaggccggtccccagaagcagcagcagcggcggcagcagccgcggcgctccggggccccctagctccatggcgcacgcacctcgcgggctctagatgcgggcggctcccggctccccgccgcttcgaggcccgtgcgcgcccaacttcatgcctcccgcgcctcgcgggccgcttcggccgccgggcccggttcgtcttctcctgtggggcgcggtgcggcggcggcgcggcagggagcgccgggctgtgggc

SEQ ID NO: 16371 - RNA, 3260 nt, Homo sapiens
  source 1..3260: mol_type = other RNA
gtccacttctgcctgccctgccaggacggagggcatgggcctgtgtggaaaccccagggctccctgactcccatgaggcttctcagggacttcctgccccgagggtcccagcatctcccaggtggaggtcctcaaggatgcccccaccagctccccacagctactgtagcaggaagtccttcttcccgaacccagagcccagggcggatctcccgggctgcgcgccaaggtggaaaccctcagggtcctgggggaaccagggcccaggtctggactccattcgggaccttcccagctccggggaatcacaacacagaagtaccccaggggctgaagccactaggcccccgtggagccctggccacctgccagagccctggccctacgcctggaaggcagagtcctggtctccagactcgctggggctgggtgttcctgtcccccgcggagggcctgcgcaggggagagctggtcccgcgtgggcctcccgattctccccacgcggaaccagctccacaaaactctgttctccaaggctccttaggcacaagacttgagttctcactaacttacccaaaacacaaccaaacacaatccctgcctggaccctctcctagcgaagcagattggagcgctgctggctcaccctcatggggcccgagaggctcaaggaccctgggggagaagttgaagcccacacaggcgcaggacacggtgggtgggagaggcggccgggcctccagaagacggggcgcttggggctgaaggggcgtgaactcccttcaagggccccttggggcggtcgggaccatcaccagatctgctgagagactgggaggagtgagttccatctgcaggggagctcaggagactcttgaactggacttagcccgagtcctgcaggtagaaggcgccgacccccacctctgctccaagccactgcctcctgaggccacagtccaactggaagcagctccacactcggtctccccagaggccgtgtccccgtccaaggccgtcttacagcagacacagaacaggaaggaaaatttggcaaacgtgtggccccacagagtccagggagaagccagcccggccccaggccggccgcatggatgctggccccgtgcacggcagccccaggccacgcaggctcccggtcccttcctagatcatgccagccagccagggcggcaggaagaggcccaccgtccccagcaggcagacgatgatgaacatccagaggaagatgcggtcgatgaccatggccacgtacttccagtcctccttcaccgagaagtctgtgtcttcggccttcaggtggtctgcaatgtactggacgccctccaccgcccgggtcagggccggcgacaggggcaggtgcgggggcggcgctttggtgctgcgggtcttgaccgtggcgctcggggacaccgaagagggctccttcttgcatgtgcatttgcacggagagggctggtctgggggtgggagctcagccgagtgggtgttgcgagaggccagggcgccggcagcctggccatctgcctcgggggcggcatcgtctcggggaacacagtactggatgctccgagaccggcaccggacgccgccttccaccgcttcgccagggctggacatgtgctggacgctgagggacctggctttggccagccctggtgcctgggtgccgtggggcgggcggcagggtccaggcgaggggtgggggctggctttctcagcttccaggggctgctgaggagggagctggtcggagggtgacttgcaggaaggcccaggctcagccggcacatccagggggacacagaaggacggtgagggcgggtgcaggctctgggtgccgctcgtggcagggggctccccttctggctcgggccagaagcgcggggcactggccatcttatgcatggactcgatgagccgccggcaattgtccttgaccacggacggccgcttcatgaggagcaggcgtggcacgatgtccaggaagaccctgcgtacccaggtgggcatggtgtgcgtgcgtggcgagcggtggtgcacgttgagcacgaagaccgtgatgacgatggacagggtgacgaagatcatggtgaacagcaggtactcgccgatgagtgggatgaccagtgaggtggacgggatgatctcggtgatgagcagcaggaagacggtgagcgacagcagcacggagatgcacagcgtgatcttctcgccacactcggagggcaggtagaagaccagcacggtgaggcaggagatgagcaggcaggggatgatgaggttgatggtgtagaagagcggcagccgccggatgacgaaggcataggtgatgtccgggtagatctcggcacagcactcgtacttcctggtgttgtaggtgcccacggcatccacgatgacccactcgccactctcccagaagtccagctggtccacgcggctgtgcatgttcaccaggtcgatcttggccttgtcgtaggtccaggagccgaatttcatggtgcagttctgctggtcgaaggggaagaaggtgacgtcgatgctgcaggagctcttgtaaatggccgggggagtccactgcacccgcccgtcatggaacaggtgggccttggtcaggtgggtgaccgcgaagtccccgtcagcattgttgtagaggacgatgtccggccgccagatgagctcggaggggatgcggatggaggtgacattctcatagtcagctgggtcccagcgcagcttgtagtcgtgccactcctggatgaggtggggcggggggaggctgcttcacccatacgttcgtggtcatcatctggttcttctcatccacgtcaatgagctgagcgatggacaggccgaagcggacgaggaccacgtccgagatgttggccacgggtcgggaccacttgttgtaaccggagaagagtttcttcaggagccgctcctcggcgtgggcccgggtctccacatggctgctggcgcgcaggaggccggtccccagaagcagcagcagcggcggcagcagccgcggcgctccggggccccctagctccatggcgcacgcacctcgcgggctctagatgcgggcggctcccggctccccgccgcttcgaggcccgtgcgcgcccaacttcatgcctcccgcgcctcgcgggccgcttcggccgccgggcccggttcgtcttctcctgtggggcgcggtgcggcggcggcgcggcagggagcgccgggctgtgggc

SEQ ID NO: 16372 - RNA, 3411 nt, Homo sapiens
  source 1..3411: mol_type = other RNA
gtccacttctgcctgccctgccaggacggagggcatgggcctgtgtggaaaccccagggctccctgactcccatgaggcttctcagggacttcctgccccgagggtcccagcatctcccaggtggaggtcctcaaggatgcccccaccagctccccacagctactgtagcaggaagtccttcttcccgaacccagagcccagggcggatctcccgggctgcgcgccaaggtggaaaccctcagggtcctgggggaaccagggcccaggtctggactccattcgggaccttcccagctccggggaatcacaacacagaagtaccccaggggctgaagccactaggcccccgtggagccctggccacctgccagagccctggccctacgcctggaaggcagagtcctggtctccagactcgctggggctgggtgttcctgtcccccgcggagggcctgcgcaggggagagctggtcccgcgtgggcctcccgattctccccacgcggaaccagctccacaaaactctgttctccaaggctccttaggcacaagacttgagttctcactaacttacccaaaacacaaccaaacacaatccctgcctggaccctctcctagcgaagcagattggagcgctgctggctcaccctcatggggcccgagaggctcaaggaccctgggggagaagttgaagcccacacaggcgcaggacacggtgggtgggagaggcggccgggcctccagaagacggggcgcttggggctgaaggggcgtgaactcccttcaagggccccttggggcggtcgggaccatcaccagatctgctgagagactgggaggagtgagttccatctgcaggggagctcaggagactcttgaactggacttagcccgagtcctgcaggtagaaggcgccgacccccacctctgctccaagccactgcctcctgaggccacagtccaactggaagcagctccacactcggtctccccagaggccgtgtccccgtccaaggccgtcttacagcagacacagaacaggaaggaaaatttggcaaacgtgtggccccacagagtccagggagaagccagcccggccccaggccggccgcatggatgctggccccgtgcacggcagccccaggccacgcaggctcccggtcccttcctagatcatgccagccagccagggcggcaggaagaggcccaccgtccccagcaggcagacgatgatgaacatccagaggaagatgcggtcgatgaccatggccacgtacttccagtcctccttcaccgagaagtctgtgtcttcggccttcaggtggtctgcaatgtactggacgccctccaccgcccgggtcagggccggcgacaggggcaggtgcgggggcggcgctttggtgctgcgggtcttgaccgtggcgctcggggacaccgaagagggctccttcttgcatgtgcatttgcacggagagggctggtctgggggtgggagctcagccgagtgggtgttgcgagaggccagggcgccggcagcctggccatctgcctcgggggcggcatcgtctcggggaacacagtactggatgctccgagaccggcaccggacgccgccttccaccgcttcgccagggctggacatgtgctggacgctgagggacctggctttggccagccctggtgcctgggtgccgtggggcgggcggcagggtccaggcgaggggtgggggctggctttctcagcttccaggggctgctgaggagggagctggtcggagggtgacttgcaggaaggcccaggctcagccggcacatccagggggacacagaaggacggtgagggcgggtgcaggctctgggtgccgctcgtggcagggggctccccttctggctcgggccagaagcgcggggcactggccatcttatgcatggactcgatgagccgccggcaattgtccttgaccacggacggccgcttcatgaggagcaggcgtggcacgatgtccaggaagaccctgcgtacccaggtgggcatggtgtgcgtgcgtggcgagcggtggtgcacgttgagcacgaagaccgtgatgacgatggacagggtgacgaagatcatggtgaacagcaggtactcgccgatgagtgggatgaccagtgaggtggacgggatgatctcggtgatgagcagcaggaagacggtgagcgacagcagcacggagatgcacagcgtgatcttctcgccacactcggagggcaggtagaagaccagcacggtgaggcaggagatgagcaggcaggggatgatgaggttgatggtgtagaagagcggcagccgccggatgacgaaggcataggtgatgtccgggtagatctcggcacagcactcgtacttcctggtgttgtaggtgcccacggcatccacgatgacccactcgccactctcccagaagtccagctggtccacgcggctgtgcatgttcaccaggtcgatcttggccttgtcgtaggtccaggagccgaatttcatggtgcagttctgctggtcgaaggggaagaaggtgacgtcgatgctgcaggagctcttgtaaatggccgggggagtccactgcacccgcccgtcatggaacaggtgggccttggtcaggtgggtgaccgcgaagtccccgtcagcattgttgtagaggactcacttgttgtagaggacgatgtccggccgccagatgagctcggaggggatgcggatggaggtgacattctcatagtcagctgggtcccagcgcagcttgtagtcgtgccactcctgcttcacccatacgttcgtggtcatcatctggttcttctcatccacgtcaatgagctgagcgatggacaggccgaagcggacgaggaccacgtccgagatgttggccacgggtcgggaccacttgttgtaaccggagaagagtttcttcaggagccgctcctcggcgtgggcccgggtctccacatggctgctggctcaggctggtccttttcgctcccatgtgaaggcaccattgccaggccaatgctggtcactctgtgatgaccaggttggagaaaagctgagaaccccaagtattgggcaaatgcagactcttgtgtcttcaaaccagaggacatttaaccctaagtcaagaggccggcttcttccaggagtcccctccctgggcattgcctggtgtccactctggagtcagctgacccggcccagccctgaggtctctcctccacctgtctggctccaggacagtgatgggcattgcaggccgctctgtcaggtggcgtttctaaccttgttctatccacagaactcgtcttcaaaaaaagtttacatgacagaaccatttagaagaaaaaaagcagagaggccttggttgaggttttggtggctctg

SEQ ID NO: 16373 - RNA, 3166 nt, Homo sapiens
  source 1..3166: mol_type = other RNA
gtccacttctgcctgccctgccaggacggagggcatgggcctgtgtggaaaccccagggctccctgactcccatgaggcttctcagggacttcctgccccgagggtcccagcatctcccaggtggaggtcctcaaggatgcccccaccagctccccacagctactgtagcaggaagtccttcttcccgaacccagagcccagggcggatctcccgggctgcgcgccaaggtggaaaccctcagggtcctgggggaaccagggcccaggtctggactccattcgggaccttcccagctccggggaatcacaacacagaagtaccccaggggctgaagccactaggcccccgtggagccctggccacctgccagagccctggccctacgcctggaaggcagagtcctggtctccagactcgctggggctgggtgttcctgtcccccgcggagggcctgcgcaggggagagctggtcccgcgtgggcctcccgattctccccacgcggaaccagctccacaaaactctgttctccaaggctccttaggcacaagacttgagttctcactaacttacccaaaacacaaccaaacacaatccctgcctggaccctctcctagcgaagcagattggagcgctgctggctcaccctcatggggcccgagaggctcaaggaccctgggggagaagttgaagcccacacaggcgcaggacacggtgggtgggagaggcggccgggcctccagaagacggggcgcttggggctgaaggggcgtgaactcccttcaagggccccttggggcggtcgggaccatcaccagatctgctgagagactgggaggagtgagttccatctgcaggggagctcaggagactcttgaactggacttagcccgagtcctgcaggtagaaggcgccgacccccacctctgctccaagccactgcctcctgaggccacagtccaactggaagcagctccacactcggtctccccagaggccgtgtccccgtccaaggccgtcttacagcagacacagaacaggaaggaaaatttggcaaacgtgtggccccacagagtccagggagaagccagcccggccccaggccggccgcatggatgctggccccgtgcacggcagccccaggccacgcaggctcccggtcccttcctagatcatgccagccagccagggcggcaggaagaggcccaccgtccccagcaggcagacgatgatgaacatccagaggaagatgcggtcgatgaccatggccacgtacttccagtcctccttcaccgagaagtctgtgtcttcggccttcaggtggtctgcaatgtactggacgccctccaccgcccgggtcagggccggcgacaggggcaggtgcgggggcggcgctttggtgctgcgggtcttgaccgtggcgctcggggacaccgaagagggctccttcttgcatgtgcatttgcacggagagggctggtctgggggtgggagctcagccgagtgggtgttgcgagaggccagggcgccggcagcctggccatctgcctcgggggcggcatcgtctcggggaacacagtactggatgctccgagaccggcaccggacgccgccttccaccgcttcgccagggctggacatgtgctggacgctgagggacctggctttggccagccctggtgcctgggtgccgtggggcgggcggcagggtccaggcgaggggtgggggctggctttctcagcttccaggggctgctgaggagggagctggtcggagggtgacttgcaggaaggcccaggctcagccggcacatccagggggacacagaaggacggtgagggcgggtgcaggctctgggtgccgctcgtggcagggggctccccttctggctcgggccagaagcgcggggcactggccatcttatgcatggactcgatgagccgccggcaattgtccttgaccacggacggccgcttcatgaggagcaggcgtggcacgatgtccaggaagaccctgcgtacccaggtgggcatggtgtgcgtgcgtggcgagcggtggtgcacgttgagcacgaagaccgtgatgacgatggacagggtgacgaagatcatggtgaacagcaggtactcgccgatgagtgggatgaccagtgaggtggacgggatgatctcggtgatgagcagcaggaagacggtgagcgacagcagcacggagatgcacagcgtgatcttctcgccacactcggagggcaggtagaagaccagcacggtgaggcaggagatgagcaggcaggggatgatgaggttgatggtgtagaagagcggcagccgccggatgacgaaggcataggtgatgtccgggtagatctcggcacagcactcgtacttcctggtgttgtaggtgcccacggcatccacgatgacccactcgccactctcccagaagtccagctggtccacgcggctgtgcatgttcaccaggtcgatcttggccttgtcgtaggtccaggagccgaatttcatggtgcagttctgctggtcgaaggggaagaaggtgacgtcgatgctgcaggagctcttgtaaatggccgggggagtccactgcacccgcccgtcatggaacaggtgggccttggtcaggtgggtgaccgcgaagtccccgtcagcattgttgtagaggactcacttgttgtagaggacgatgtccggccgccagatgagctcggaggggatgcggatggaggtgacattctcatagtcagctgggtcccagcgcagcttgtagtcgtgccactcctgcttcacccatacgttcgtggtcatcatctggttcttctcatccacgtcaatgagctgagcgatggacaggccgaagcggacgaggaccacgtccgagatgttggccacgggtcgggaccacttgttgtaaccggagaagagtttcttcaggagccgctcctcggcgtgggcccgggtctccacatggctgctggctcgcgggctctagatgcgggcggctcccggctccccgccgcttcgaggcccgtgcgcgcccaacttcatgcctcccgcgcctcgcgggccgcttcggccgccgggcccggttcgtcttctcctgtggggcgcggtgcggcggcggcgcggcagggagcgccgggctgtgggc

SEQ ID NO: 16374 - RNA, 5942 nt, Homo sapiens
  source 1..5942: mol_type = other RNA
gtccacttctgcctgccctgcccacgcactgccattccacagtgtacagatggggaaactgaggcacggtacagggacatggtttccccccttcctggagccaggacccatttctttctccacctggaaaggtgggcagcaggaaaacaccacacacctctgctttgagataaaaaaaaactgctggctgctggcactgccaggaaaggcagccccagcactccaggcccctccacaatgtgctgggcggctccccatggagggctaccgagtacagttccttcagagcatttgggttgggtgggctggcagaggggacaggtcagaaggtgaggccgggccgagccacgtcttccatccatcttggaggcagaaagaggccacttccagagctcctggggtctgaggccatgtgagagacgccggccatacagcagcagatgccagacctctccctgtctgcacgcagggatgccggagtgcagagccaggaccagctctgtacaaataagtaacagtctagctatcagacctgccccgtaaggaagtggccaccccatgtgggagttccttgtccctggaaaggtccaaacagaaaccacgggaccccatctcagaggagctacgtgcaaacatttgctctatgtgaaatatatttgttacagtattcaaccttaaaatggaaggaacggccggcacaccatgacagggagcaccttgagggcgttgtgctcagtggaataagccggtcacaaaaggacaaatcctgtaggagtctatcgtacgaggtccctagagtcaaactcatagagacagagagaagggcaggtgccaggggctgcgggaaggggagcggttggcgtttaaaggggacagggcttcagtctgagaagaaaggctccacgggtggagggtactgagggctgcgcagcattgtgaatgtgcttagtgacaccgaactgtgcatgtgaaatggttaaaatgctaagttttatgtcatgttatcaattacatttttaagaatgcatccatcgtcacccgcccgtactgtgaatgagagacgctgtccctgctttcgagacttatggtctgaggggagaggcagcctggaaagtggcaattaggatgcccagaggggagagagagcagcaaagagtgagggtgtcctgggagggcacagaagaggaaccaagagcggggcgggctcccaggaaggagtgagtgccagtcccaggtcggagtaaggggccactctggcaaaaaccacatccaaaagcccagaggagacagaagctgcacatctggggacctgaaagcaaacccagagggccagtgtcacagacagaatgggcagagtgggaggaggcctcatcccagagcatccacgccttggaaagcaggtgcccctgggagccaggcaggtccacgctgccttcccacctaacaaaggaaacaaatgaacaaaccccagctcccgaggggccaggccctgggcactccattccccagcatcacctgactcagtcctcaagatccccccaaaaacgcccataacagtgggtatattactcccattttacagatgaggaaactgcagcctgatggaggtgagctccgcctcgatgcaggaagtgttttatgacagtgcggtagaattttaaaacaaaagaacacgcgatcaggcgtgcactgtgccacccacgctgaccgagatgcgtcgacttctcacagcacagattcctctgctgactctaaacccaggagcttctgagccctcagccctaaaccagagcagccactctgagctgagtgtctcctctgcatccggcacgatttcagacttgacgggggtgcagagaaaatgtgaggcgtcacttccgcccctcaaaaactgacattttaaatgagaggtgcagagtctcatgtgtgggaaaaattggaacaatcgtgggactgttgctttaaaacagcccctggtccacggttccccatctcagggcttataagagaacaaggctcacagagcattggaagctaggacaggtatgagtgtgtgtcgcctacaaagtgattccaaacgcagtgaggtagagagatgaagccagcccgccaggatgaacacagggaaggaggtgcttcatctcctctctcacgtcccaaaatagaaaaatgcttttttccccaccagaagacggggtctgcctcctatgcactgacactgccttctcttcccactcatcagtcttcaaaacccaccgggagtggggacagttgagctggaggtgagccctgcattcagaaggcagcatcctgccctggaccacggccctgttcacactgggtatacagcaggcgttttgtctgacacttcatccattcagtgggtcgggaaacagggctgaggatgaggaagaggaagcccagcaaccggggccttggaaaattgcggcaggacgaatcaaacacaaccgcatctcataaggctgggagggagggtgccccatgaaaatgatttctccagccgcccgcccgaagggtatttttagcaactgtcgcatgcccaccatgggcaagccaggctgatgagaaagacagcgggaactggagaatggaatgatggcaacgaaataaaaccacgcgtggatcaaaactgccaagttcccagtaacttgaagaagtgcacttcagaggaccaggcctcacgcagctccggctgagtttgtgagcccggtgatgcagcagcaccctggcctccacgcccggaaggaacatgttggtgccaggccacctttcccgttcctgaaggtcgcagaagggccttctcaaatcaatgggcagacaatgctatcctcaggaacaactttgaaaagctgacttgaacatgagccccaaaccctgagggatgaatcaaagctaagaattcaagactagggaagttactgggaccccagactcaagaatcaggccatcgctggtgcagggtaggggcaagaaggatggggtgtggtggggagttctgcccccatgacttccccgccctgcttttcttgggcttggttccttccttgattctacaaaatgtgctttggaccaatcagtgaaacgatattaaattgtccattttgtaggttaaaattctatagggttcaacctaatatttggctttgcggttcagagagactctctttccgcatctgattcttcagcattgtacctggcaccagagccttccacatgccaagctgttgcaggctgggcccccatccaggagcaattactgaacgaaacacttctttttccccttaaaaagactcgtgaagccacaccatgccactgttattgccaaggtgcttgagcgatgattttccacatgcttgtggccgtaacttacatttaatgacatgagtcaggggcttgtttctgcaccagaagaccaataagcctcccggtgacagatagggtctgtcaccccattcgtcaaactctacgtcatgtcacctcatgatattcccaatgatgccttacagtcgccatatgcacaacggcctccgtagtacgcagctgagtgtgaaacatatggagagagtaaaaggctgtgctaatgtctgctggagtcaacgattcctaagtggagggtctgtgccattttgcttttccttctttcttataattttctgcagattcttcattttctacagggcatgtctcactccgttcagctttctgtaacaaaataccatagactgggtggcttataaacaacaggaatctatttctctcagttctggaggctggaagtccaagattaaggtgcctgcagatttggtgtctggtgaagccacctccccattggacagccgtctgtctttttgctgggtggcatgtggcagagggggtgaggggtctctccctggcctctttcataaggaaactaattccattcatgacctaatcacctccccttgtcctagcatcatcagcctggggatgaggtttcacctcccctcctcctagtatcaccagcctggggatgaggattcacctcccctcctcctagtatcaccagcctgaggacgaggattcaccttccctcctcctagcatcaccagcctggggacgagtattcacctcccctcctcctagtatcatcagcctggggatgaggattcacctcccctcctcctagtatcaccagcctgaggatgaggattcacctcccctcctcctagtatcatcagcctggggacgagtattcacctcccctcctcctagcatcatcagcctggggactaggatttcaacatctgagcttgggggacagaaacagcccgtagcaaagcatgtgcatttttatcatggaaaacgtgtttttcaaatttgaatcagcattttgtctacatgatggcatagacaccgggggtccccacctggtccccagcactggcggctgcaccgtcgccagctcctgggagtgaggtctgacagcttgcagccactccattccccagatagctgagtctggccacagggagctgctgctcctggggagctgtcctcccaccagtgaaggcctcgccagtgactgaccacgtggaggcacagaaggcgtcccctggcctcagggcaggcccaccccagggtgcagctcccactccggagcacctgtgggggaccagaccacggtgcaactcgagctgaggtcacctccctgctcagccccttcacccacccggtcctgctccccaccctctgtcctgaggaaaccccaataaatcatgtgatgtgatgagaattatgtcactgccacaggactgctgtgagaatcgtgaagtaaaggggctggcacctggtacactgaggggctcaccaaactccagcgtcccagcactgtggggctccagccggccaggcatctgataggcagcgccttggcattccagaagggcggctgtgaacacggggttcagagcctgcacactggcagaggcgtctgcaccatagaccgagccaggtgccggggcagagcacaagcagcctgtcctcgctccaagaccccaattccccttctcctgtcagtgggaacctaggtcccaggctctctgtggagccccatgctgcaaaatatcttagtcggcgccctgttcctgtcaggcccaggttctggggagagcaggggtgggagagggcgctgggtgctggccagggcagtgcacacagttgtctgtcctggccgtagggcagtgaccctgttcccaccacaggcggccctggcaggcaggcaaaccaccaacagaccccaggccctgcacctgacgtctgctctggaagtcggtctgcatttagttttgggtttaacaaacatttttaaccccatcattttcaacgagtgtaagattcacaaaagcattggaagttctattaaaaagaggctcaaaattactacagaaaccaaaggacagagttttaaaaatagcaactggtgagaaaaatgacaaatgccgcacatttgatggggtgagtcatctcctggcggcgccatcctcagccacacccgagtgaagggctgcgcctgatgctgtcctcagggaccagctggacagggacgcggggacgtgcttctctatgtgcggggagaggcgggcgtaggcggctggcgctggctccccgacggcaaaccaaggagcttaaaggccaggcagggacaaggggttgctgaggaaacttccggggcttctcaggtccaggctgaccaggtttacacaccagaaagtgagggccccgcacagggcagggatcctcggccagggcgaggtgggcagggcagggctgccccatgtggacattcattcattcctacccacgcctgccacacattcattcattcatttccacctgcacccatcacacatccattccttccctcccccgcccaccacattcat

SEQ ID NO: 16375 - RNA, 5470 nt, Homo sapiens
  source 1..5470: mol_type = other RNA
gtccacttctgcctgccctgcccacgcactgccattccacagtgtacagatggggaaactgaggcacggtacagggacatggtttccccccttcctggagccaggacccatttctttctccacctggaaaggtgggcagcaggaaaacaccacacacctctgctttgagataaaaaaaaactgctggctgctggcactgccaggaaaggcagccccagcactccaggcccctccacaatgtgctgggcggctccccatggagggctaccgagtacagttccttcagagcatttgggttgggtgggctggcagaggggacaggtcagaaggtgaggccgggccgagccacgtcttccatccatcttggaggcagaaagaggccacttccagagctcctggggtctgaggccatgtgagagacgccggccatacagcagcagatgccagacctctccctgtctgcacgcagggatgccggagtgcagagccaggaccagctctgtacaaataagtaacagtctagctatcagacctgccccgtaaggaagtggccaccccatgtgggagttccttgtccctggaaaggtccaaacagaaaccacgggaccccatctcagaggagctacgtgcaaacatttgctctatgtgaaatatatttgttacagtattcaaccttaaaatggaaggaacggccggcacaccatgacagggagcaccttgagggcgttgtgctcagtggaataagccggtcacaaaaggacaaatcctgtaggagtctatcgtacgaggtccctagagtcaaactcatagagacagagagaagggcaggtgccaggggctgcgggaaggggagcggttggcgtttaaaggggacagggcttcagtctgagaagaaaggctccacgggtggagggtactgagggctgcgcagcattgtgaatgtgcttagtgacaccgaactgtgcatgtgaaatggttaaaatgctaagttttatgtcatgttatcaattacatttttaagaatgcatccatcgtcacccgcccgtactgtgaatgagagacgctgtccctgctttcgagacttatggtctgaggggagaggcagcctggaaagtggcaattaggatgcccagaggggagagagagcagcaaagagtgagggtgtcctgggagggcacagaagaggaaccaagagcggggcgggctcccaggaaggagtgagtgccagtcccaggtcggagtaaggggccactctggcaaaaaccacatccaaaagcccagaggagacagaagctgcacatctggggacctgaaagcaaacccagagggccagtgtcacagacagaatgggcagagtgggaggaggcctcatcccagagcatccacgccttggaaagcaggtgcccctgggagccaggcaggtccacgctgccttcccacctaacaaaggaaacaaatgaacaaaccccagctcccgaggggccaggccctgggcactccattccccagcatcacctgactcagtcctcaagatccccccaaaaacgcccataacagtgggtatattactcccattttacagatgaggaaactgcagcctgatggaggtgagctccgcctcgatgcaggaagtgttttatgacagtgcggtagaattttaaaacaaaagaacacgcgatcaggcgtgcactgtgccacccacgctgaccgagatgcgtcgacttctcacagcacagattcctctgctgactctaaacccaggagcttctgagccctcagccctaaaccagagcagccactctgagctgagtgtctcctctgcatccggcacgatttcagacttgacgggggtgcagagaaaatgtgaggcgtcacttccgcccctcaaaaactgacattttaaatgagaggtgcagagtctcatgtgtgggaaaaattggaacaatcgtgggactgttgctttaaaacagcccctggtccacggttccccatctcagggcttataagagaacaaggctcacagagcattggaagctaggacaggtatgagtgtgtgtcgcctacaaagtgattccaaacgcagtgaggtagagagatgaagccagcccgccaggatgaacacagggaaggaggtgcttcatctcctctctcacgtcccaaaatagaaaaatgcttttttccccaccagaagacggggtctgcctcctatgcactgacactgccttctcttcccactcatcagtcttcaaaacccaccgggagtggggacagttgagctggaggtgagccctgcattcagaaggcagcatcctgccctggaccacggccctgttcacactgggtatacagcaggcgttttgtctgacacttcatccattcagtgggtcgggaaacagggctgaggatgaggaagaggaagcccagcaaccggggccttggaaaattgcggcaggacgaatcaaacacaaccgcatctcataaggctgggagggagggtgccccatgaaaatgatttctccagccgcccgcccgaagggtatttttagcaactgtcgcatgcccaccatgggcaagccaggctgatgagaaagacagcgggaactggagaatggaatgatggcaacgaaataaaaccacgcgtggatcaaaactgcctgggaacagaaacatacagaactgatgctgaagaagacaaaatatgtgacgcggagaatgaagcggggaaggagggagcccgggcatggcaggaaggggcagggagctgggcagcaggtgctccccagaggaaagagaggcagggtggggagcaggtgaggaggaggaggaagcgctgaactttcctgagctgcggaggcgggcggggtcgggggtggtttggggacaaaccaagttcccagtaacttgaagaagtgcacttcagaggaccaggcctcacgcagctccggctgagtttgtgagcccggtgatgcagcagcaccctggcctccacgcccggaaggaacatgttggtgccaggccacctttcccgttcctgaaggtcgcagaagggccttctcaaatcaatgggcagacaatgctatcctcaggaacaactttgaaaagctgacttgaacatgagccccaaaccctgagggatgaatcaaagctaagaattcaagactagggaagttactgggaccccagactcaagaatcaggccatcgctggtgcagggtaggggcaagaaggatggggtgtggtggggagttctgcccccatgacttccccgccctgcttttcttgggcttggttccttccttgattctacaaaatgtgctttggaccaatcagtgaaacgatattaaattgtccattttgtaggttaaaattctatagggttcaacctaatatttggctttgcggttcagagagactctctttccgcatctgattcttcagcattgtacctggcaccagagccttccacatgccaagctgttgcaggctgggcccccatccaggagcaattactgaacgaaacacttctttttccccttaaaaagactcgtgaagccacaccatgccactgttattgccaaggtgcttgagcgatgattttccacatgcttgtggccgtaacttacatttaatgacatgagtcaggggcttgtttctgcaccagaagaccaataagcctcccggtgacagatagggtctgtcaccccattcgtcaaactctacgtcatgtcacctcatgatattcccaatgatgccttacagtcgccatatgcacaacggcctccgtagtacgcagctgagtgtgaaacatatggagagagtaaaaggctgtgctaatgtctgctggagtcaacgattcctaagtggagggtctgtgccattttgcttttccttctttcttataattttctgcagattcttcattttctacagggcatgtctcactccgttcagctttctggtccccagcactggcggctgcaccgtcgccagctcctgggagtgaggtctgacagcttgcagccactccattccccagatagctgagtctggccacagggagctgctgctcctggggagctgtcctcccaccagtgaaggcctcgccagtgactgaccacgtggaggcacagaaggcgtcccctggcctcagggcaggcccaccccagggtgcagctcccactccggagcacctgtgggggaccagaccacggtgcaactcgagctgaggtcacctccctgctcagccccttcacccacccggtcctgctccccaccctctgtcctgaggaaaccccaataaatcatgtgatgtgatgagaattatgtcactgccacaggactgctgtgagaatcgtgaagtaaaggggctggcacctggtacactgaggggctcaccaaactccagcgtcccagcactgtggggctccagccggccaggcatctgataggcagcgccttggcattccagaagggcggctgtgaacacggggttcagagcctgcacactggcagaggcgtctgcaccatagaccgagccaggtgccggggcagagcacaagcagcctgtcctcgctccaagaccccaattccccttctcctgtcagtgggaacctaggtcccaggctctctgtggagccccatgctgcaaaatatcttagtcggcgccctgttcctgtcaggcccaggttctggggagagcaggggtgggagagggcgctgggtgctggccagggcagtgcacacagttgtctgtcctggccgtagggcagtgaccctgttcccaccacaggcggccctggcaggcaggcaaaccaccaacagaccccaggccctgcacctgacgtctgctctggaagtcggtctgcatttagttttgggtttaacaaacatttttaaccccatcattttcaacgagtgtaagattcacaaaagcattggaagttctattaaaaagaggctcaaaattactacagaaaccaaaggacagagttttaaaaatagcaactggtgagaaaaatgacaaatgccgcacatttgatggggtgagtcatctcctggcggcgccatcctcagccacacccgagtgaagggctgcgcctgatgctgtcctcagggaccagctggacagggacgcggggacgtgcttctctatgtgcggggagaggcgggcgtaggcggctggcgctggctccccgacggcaaaccaaggagcttaaaggccaggcagggacaaggggttgctgaggaaacttccggggcttctcaggtccaggctgaccaggtttacacaccagaaagtgagggccccgcacagggcagggatcctcggccagggcgaggtgggcagggcagggctgccccatgtggacattcattcattcctacccacgcctgccacacattcattcattcatttccacctgcacccatcacacatccattccttccctcccccgcccaccacattcat

SEQ ID NO: 16376 - RNA, 6174 nt, Homo sapiens
  source 1..6174: mol_type = other RNA
gtccacttctgcctgccctgcccacgcactgccattccacagtgtacagatggggaaactgaggcacggtacagggacatggtttccccccttcctggagccaggacccatttctttctccacctggaaaggtgggcagcaggaaaacaccacacacctctgctttgagataaaaaaaaactgctggctgctggcactgccaggaaaggcagccccagcactccaggcccctccacaatgtgctgggcggctccccatggagggctaccgagtacagttccttcagagcatttgggttgggtgggctggcagaggggacaggtcagaaggtgaggccgggccgagccacgtcttccatccatcttggaggcagaaagaggccacttccagagctcctggggtctgaggccatgtgagagacgccggccatacagcagcagatgccagacctctccctgtctgcacgcagggatgccggagtgcagagccaggaccagctctgtacaaataagtaacagtctagctatcagacctgccccgtaaggaagtggccaccccatgtgggagttccttgtccctggaaaggtccaaacagaaaccacgggaccccatctcagaggagctacgtgcaaacatttgctctatgtgaaatatatttgttacagtattcaaccttaaaatggaaggaacggccggcacaccatgacagggagcaccttgagggcgttgtgctcagtggaataagccggtcacaaaaggacaaatcctgtaggagtctatcgtacgaggtccctagagtcaaactcatagagacagagagaagggcaggtgccaggggctgcgggaaggggagcggttggcgtttaaaggggacagggcttcagtctgagaagaaaggctccacgggtggagggtactgagggctgcgcagcattgtgaatgtgcttagtgacaccgaactgtgcatgtgaaatggttaaaatgctaagttttatgtcatgttatcaattacatttttaagaatgcatccatcgtcacccgcccgtactgtgaatgagagacgctgtccctgctttcgagacttatggtctgaggggagaggcagcctggaaagtggcaattaggatgcccagaggggagagagagcagcaaagagtgagggtgtcctgggagggcacagaagaggaaccaagagcggggcgggctcccaggaaggagtgagtgccagtcccaggtcggagtaaggggccactctggcaaaaaccacatccaaaagcccagaggagacagaagctgcacatctggggacctgaaagcaaacccagagggccagtgtcacagacagaatgggcagagtgggaggaggcctcatcccagagcatccacgccttggaaagcaggtgcccctgggagccaggcaggtccacgctgccttcccacctaacaaaggaaacaaatgaacaaaccccagctcccgaggggccaggccctgggcactccattccccagcatcacctgactcagtcctcaagatccccccaaaaacgcccataacagtgggtatattactcccattttacagatgaggaaactgcagcctgatggaggtgagctccgcctcgatgcaggaagtgttttatgacagtgcggtagaattttaaaacaaaagaacacgcgatcaggcgtgcactgtgccacccacgctgaccgagatgcgtcgacttctcacagcacagattcctctgctgactctaaacccaggagcttctgagccctcagccctaaaccagagcagccactctgagctgagtgtctcctctgcatccggcacgatttcagacttgacgggggtgcagagaaaatgtgaggcgtcacttccgcccctcaaaaactgacattttaaatgagaggtgcagagtctcatgtgtgggaaaaattggaacaatcgtgggactgttgctttaaaacagcccctggtccacggttccccatctcagggcttataagagaacaaggctcacagagcattggaagctaggacaggtatgagtgtgtgtcgcctacaaagtgattccaaacgcagtgaggtagagagatgaagccagcccgccaggatgaacacagggaaggaggtgcttcatctcctctctcacgtcccaaaatagaaaaatgcttttttccccaccagaagacggggtctgcctcctatgcactgacactgccttctcttcccactcatcagtcttcaaaacccaccgggagtggggacagttgagctggaggtgagccctgcattcagaaggcagcatcctgccctggaccacggccctgttcacactgggtatacagcaggcgttttgtctgacacttcatccattcagtgggtcgggaaacagggctgaggatgaggaagaggaagcccagcaaccggggccttggaaaattgcggcaggacgaatcaaacacaaccgcatctcataaggctgggagggagggtgccccatgaaaatgatttctccagccgcccgcccgaagggtatttttagcaactgtcgcatgcccaccatgggcaagccaggctgatgagaaagacagcgggaactggagaatggaatgatggcaacgaaataaaaccacgcgtggatcaaaactgcctgggaacagaaacatacagaactgatgctgaagaagacaaaatatgtgacgcggagaatgaagcggggaaggagggagcccgggcatggcaggaaggggcagggagctgggcagcaggtgctccccagaggaaagagaggcagggtggggagcaggtgaggaggaggaggaagcgctgaactttcctgagctgcggaggcgggcggggtcgggggtggtttggggacaaaccaagttcccagtaacttgaagaagtgcacttcagaggaccaggcctcacgcagctccggctgagtttgtgagcccggtgatgcagcagcaccctggcctccacgcccggaaggaacatgttggtgccaggccacctttcccgttcctgaaggtcgcagaagggccttctcaaatcaatgggcagacaatgctatcctcaggaacaactttgaaaagctgacttgaacatgagccccaaaccctgagggatgaatcaaagctaagaattcaagactagggaagttactgggaccccagactcaagaatcaggccatcgctggtgcagggtaggggcaagaaggatggggtgtggtggggagttctgcccccatgacttccccgccctgcttttcttgggcttggttccttccttgattctacaaaatgtgctttggaccaatcagtgaaacgatattaaattgtccattttgtaggttaaaattctatagggttcaacctaatatttggctttgcggttcagagagactctctttccgcatctgattcttcagcattgtacctggcaccagagccttccacatgccaagctgttgcaggctgggcccccatccaggagcaattactgaacgaaacacttctttttccccttaaaaagactcgtgaagccacaccatgccactgttattgccaaggtgcttgagcgatgattttccacatgcttgtggccgtaacttacatttaatgacatgagtcaggggcttgtttctgcaccagaagaccaataagcctcccggtgacagatagggtctgtcaccccattcgtcaaactctacgtcatgtcacctcatgatattcccaatgatgccttacagtcgccatatgcacaacggcctccgtagtacgcagctgagtgtgaaacatatggagagagtaaaaggctgtgctaatgtctgctggagtcaacgattcctaagtggagggtctgtgccattttgcttttccttctttcttataattttctgcagattcttcattttctacagggcatgtctcactccgttcagctttctgtaacaaaataccatagactgggtggcttataaacaacaggaatctatttctctcagttctggaggctggaagtccaagattaaggtgcctgcagatttggtgtctggtgaagccacctccccattggacagccgtctgtctttttgctgggtggcatgtggcagagggggtgaggggtctctccctggcctctttcataaggaaactaattccattcatgacctaatcacctccccttgtcctagcatcatcagcctggggatgaggtttcacctcccctcctcctagtatcaccagcctggggatgaggattcacctcccctcctcctagtatcaccagcctgaggacgaggattcaccttccctcctcctagcatcaccagcctggggacgagtattcacctcccctcctcctagtatcatcagcctggggatgaggattcacctcccctcctcctagtatcaccagcctgaggatgaggattcacctcccctcctcctagtatcatcagcctggggacgagtattcacctcccctcctcctagcatcatcagcctggggactaggatttcaacatctgagcttgggggacagaaacagcccgtagcaaagcatgtgcatttttatcatggaaaacgtgtttttcaaatttgaatcagcattttgtctacatgatggcatagacaccgggggtccccacctggtccccagcactggcggctgcaccgtcgccagctcctgggagtgaggtctgacagcttgcagccactccattccccagatagctgagtctggccacagggagctgctgctcctggggagctgtcctcccaccagtgaaggcctcgccagtgactgaccacgtggaggcacagaaggcgtcccctggcctcagggcaggcccaccccagggtgcagctcccactccggagcacctgtgggggaccagaccacggtgcaactcgagctgaggtcacctccctgctcagccccttcacccacccggtcctgctccccaccctctgtcctgaggaaaccccaataaatcatgtgatgtgatgagaattatgtcactgccacaggactgctgtgagaatcgtgaagtaaaggggctggcacctggtacactgaggggctcaccaaactccagcgtcccagcactgtggggctccagccggccaggcatctgataggcagcgccttggcattccagaagggcggctgtgaacacggggttcagagcctgcacactggcagaggcgtctgcaccatagaccgagccaggtgccggggcagagcacaagcagcctgtcctcgctccaagaccccaattccccttctcctgtcagtgggaacctaggtcccaggctctctgtggagccccatgctgcaaaatatcttagtcggcgccctgttcctgtcaggcccaggttctggggagagcaggggtgggagagggcgctgggtgctggccagggcagtgcacacagttgtctgtcctggccgtagggcagtgaccctgttcccaccacaggcggccctggcaggcaggcaaaccaccaacagaccccaggccctgcacctgacgtctgctctggaagtcggtctgcatttagttttgggtttaacaaacatttttaaccccatcattttcaacgagtgtaagattcacaaaagcattggaagttctattaaaaagaggctcaaaattactacagaaaccaaaggacagagttttaaaaatagcaactggtgagaaaaatgacaaatgccgcacatttgatggggtgagtcatctcctggcggcgccatcctcagccacacccgagtgaagggctgcgcctgatgctgtcctcagggaccagctggacagggacgcggggacgtgcttctctatgtgcggggagaggcgggcgtaggcggctggcgctggctccccgacggcaaaccaaggagcttaaaggccaggcagggacaaggggttgctgaggaaacttccggggcttctcaggtccaggctgaccaggtttacacaccagaaagtgagggccccgcacagggcagggatcctcggccagggcgaggtgggcagggcagggctgccccatgtggacattcattcattcctacccacgcctgccacacattcattcattcatttccacctgcacccatcacacatccattccttccctcccccgcccaccacattcat

SEQ ID NO: 16377 - RNA, 2490 nt, Homo sapiens
  source 1..2490: mol_type = other RNA
gtccacttctgcctgccctgccctaccctccccctttgggtttgtttgaggtttcattccacaaataagcagcagataaaatactttacaaggtacagcacagttgtattgaagaaaaaaaggacccaactcttactttaggagtattaggcctggacttcccctgccccatgcaataaagcaagttttatatacactccccatatttttttctaacattttcttatataaatttaaatattttacaaaaaaaggcttttttcctccaaacatataaatctgagtgaaacatagattccccacccgagaacttgtttcttcactaaaatataaatgttgtctgatattaagggtaaatgtcttttgaccactggagatcactgaagtctgaattgcaccgtggagaaggcacttgtgttttctgaggtctccagcaagtatctcagtgagcactcatagaattgctgtctgtcctccagaacccgtgccaaggcctccgagtgcccagttactgaggcagctggggaaaaacgttgagtaaacatgattctacaattacggagataaaaaataaaaacagcatggactggttctaccctagaatcaaactacaacaaaatccaaagtgttcattcatgtagattcaaaatgacttcattctgtcataaattataaaatacaaaggtggctgttttaatgacaaaactcaaaacagtactaaaaggggtttgtgtcaatggacaaaagtcagtccctctaggtagggccccaaggagcatcacccaggttgaagggtggttttcctactgctgggccagaagtgctgtcctattggccttcatcttctccagccgcttggccaggtggctgttggtcatctccatctcctcaatcttgtccagtgctgttcgtaactctcgttgtagcttccgtttttctgctttcaattcatcttcaactttctcagcattctcagcagcagttttatatctcagaacctgtccctcaagccggctaatactttgctccaaggtagttatatcctgttctgcttttgaaagcttaaatttgtattcgctaatttgtctattggcatctctctgcatttcgatgaactgcaagtctgagccattctgcagtcctgccaggtcacccactgtgccatcattcctggagcatttctgtcgttcctcctctaactgaagcttcagttttctaatctgtgacagtagttcttccttctctccagcaagttttcgtagccttacatctaatggcccttctcctgctgactccaagacctgagcagcttcctgagacacaacagtgatggctccagccactggttcatgactgacatcaccattgggagtgccatcggggattataactaagccatgtttcccaatttttttatctttccaaagaagtgtctcctggaggtcaaacacctcttttgtcatggtgtctattttctgctgcatgcgctgcttctcctcaataagctcatctctttgccgcaggccttctttaagttcttccatcttatgctgcagcacactacacatatgtttctgcctttctaactcctttgatttttcttcattttctctataaaattctgccatctgttcctcctgctcttcaataacatccttgagtgtgtctacttggtagatcaaattgttcttctcattgtctaactgtgcattggaaaccatggctttcttgtatttttcttccacttcagacaaagattcccgcaattcacttaatgaagtgtctggatctattaagctgctggtgtccccacttcctcgtctggatgagtttccacttagaggggttgttgctgaggcagaatttcgagatgaaggtcttgtataattttcagcatactgtttgtcagatttttcatccaaagttcgaggaccataagggttatataatccaccattgtacaatgatgccagtaggtctttatgagaatcagaagacctcttcttcattccatgagagtgactgtaagaatgattcctgtgactgccaacacttcgaatggacaatgcatcctcaactcccagataaggacgatggtgactggaccggtgggaatacctggccctttccgaatcttcctctttttgttgtcgttccagttctctcatgcgtatatctcttgcttctgcccgggcagcccgttttgctgccagccttgcctctgcctctctggcaatgttactcaaagcttcatcttctgcagaaaatcggtctttcacaggtgttcttttccttccagaagcaggagtccccatcttgtgttcttaatagtcttttaactttgaaagtgatttaactgtgttttcagcccttagtgatggtagctctcctttccactgacatttacatctagaccccttcatttatcttcccacatcccgctctccttctctcttgtttcattactacatccacattctcttcccatta

SEQ ID NO: 16378 - RNA, 2498 nt, Homo sapiens
  source 1..2498: mol_type = other RNA
gtccacttctgcctgccctgccctaccctccccctttgggtttgtttgaggtttcattccacaaataagcagcagataaaatactttacaaggtacagcacagttgtattgaagaaaaaaaggacccaactcttactttaggagtattaggcctggacttcccctgccccatgcaataaagcaagttttatatacactccccatatttttttctaacattttcttatataaatttaaatattttacaaaaaaaggcttttttcctccaaacatataaatctgagtgaaacatagattccccacccgagaacttgtttcttcactaaaatataaatgttgtctgatattaagggtaaatgtcttttgaccactggagatcactgaagtctgaattgcaccgtggagaaggcacttgtgttttctgaggtctccagcaagtatctcagtgagcactcatagaattgctgtctgtcctccagaacccgtgccaaggcctccgagtgcccagttactgaggcagctggggaaaaacgttgagtaaacatgattctacaattacggagataaaaaataaaaacagcatggactggttctaccctagaatcaaactacaacaaaatccaaagtgttcattcatgtagattcaaaatgacttcattctgtcataaattataaaatacaaaggtggctgttttaatgacaaaactcaaaacagtactaaaaggggtttgtgtcaatggacaaaagtcagtccctctaggtagggccccaaggagcatcacccaggttgaagggtggttttcctactgctgggccagaagtgctgtcctattggccttcatcttctccagccgcttggccaggtggctgttggtcatctccatctcctcaatcttgtccagtgctgttcgtaactctcgttgtagcttccgtttttctgctttcaattcatcttcaactttctcagcattctcagcagcagttttatatctcagaacctgtccctcaagccggctaatactttgctccaaggtagttatatcctgttctgcttttgaaagcttaaatttgtattcgctaatttgtctattggcatctctctgcatttcgatgaactgcaagtctgagccattctgcagtcctgccaggtcacccactgtgccatcattcctggagcatttctgtcgttcctcctctaactgaagcttcagttttctaatctgtgacagtagttcttccttctctccagcaagttttcgtagccttacatctaatggcccttctcctgctgactccaagacctgagcagcttcctgagacacaacagtgatggctccagccactggttcatgactgacatcaccattgggagtgccatcggggattataactaagccatgtttctcaataagctcatctctttgccgcaggccttctttaagttcttccatcttatgctgcagcacactacacatatgtttctgcctttctaactcctttgatttttcttcattttctctataaaattctgccatctgttcctcctgctcttcaataacatccttgagtgtgtctacttggtagatcaaattgttcttctcattgtctaactgtgcattggaaaccatggctttcttgtatttttcttccacttcagacaaagattcccgcaattcacttaatgaagtgtctggatctattaagctgctggtgtccccacttcctcgtctggatgagtttccacttagaggggttgttgctgaggcagaatttcgagatgaaggtcttgtataattttcagcatactgtttgtcagatttttcatccaacctgtgactgccaacacttcgaatggacaatgcatcctcaactcccagataaggacgatggtgactggaccggtgggaatacctggccctttccgaatcttcctctttttgttgtcgttccagttctctcatgcgtatatctcttgcttctgcccgggcagcccgttttgctgccagccttgcctctgcctctctggcaatgttactcaaagcttcatcttctgcagaaaatcggtctttcacaggtgttcttttccttccagaagcaggagtccccatcttgtgttcttaatagtcttttaactttgaaagtgatttaactgtgttttcagcccttagtgatggtagctctcctttccactgacatttacatctagaccccttcatttatcttcccacatctgtgttagggcgcgcgctgcgactgcgtcgctgtccgggaagggccgaagagctgctcgcccgcccggcgcccgctggggctatgggcgaggggcgcagctggacgactcagtcctgggtccccggccaggcgggcggggatggacgcggcggctcccggcactggcagccggctagtcggtcaggccgatgtgccctctgcgccgcggctgagacagcgggaaccggccccgggaggagccgcagcctgagcggccgactgaggag

SEQ ID NO: 16379 - RNA, 2429 nt, Homo sapiens
  source 1..2429: mol_type = other RNA
gtccacttctgcctgccctgccctaccctccccctttgggtttgtttgaggtttcattccacaaataagcagcagataaaatactttacaaggtacagcacagttgtattgaagaaaaaaaggacccaactcttactttaggagtattaggcctggacttcccctgccccatgcaataaagcaagttttatatacactccccatatttttttctaacattttcttatataaatttaaatattttacaaaaaaaggcttttttcctccaaacatataaatctgagtgaaacatagattccccacccgagaacttgtttcttcactaaaatataaatgttgtctgatattaagggtaaatgtcttttgaccactggagatcactgaagtctgaattgcaccgtggagaaggcacttgtgttttctgaggtctccagcaagtatctcagtgagcactcatagaattgctgtctgtcctccagaacccgtgccaaggcctccgagtgcccagttactgaggcagctggggaaaaacgttgagtaaacatgattctacaattacggagataaaaaataaaaacagcatggactggttctaccctagaatcaaactacaacaaaatccaaagtgttcattcatgtagattcaaaatgacttcattctgtcataaattataaaatacaaaggtggctgttttaatgacaaaactcaaaacagtactaaaaggggtttgtgtcaatggacaaaagtcagtccctctaggtagggccccaaggagcatcacccaggttgaagggtggttttcctactgctgggccagaagtgctgtcctattggccttcatcttctccagccgcttggccaggtggctgttggtcatctccatctcctcaatcttgtccagtgctgttcgtaactctcgttgtagcttccgtttttctgctttcaattcatcttcaactttctcagcattctcagcagcagttttatatctcagaacctgtccctcaagccggctaatactttgctccaaggtagttatatcctgttctgcttttgaaagcttaaatttgtattcgctaatttgtctattggcatctctctgcatttcgatgaactgcaagtctgagccattctgcagtcctgccaggtcacccactgtgccatcattcctggagcatttctgtcgttcctcctctaactgaagcttcagttttctaatctgtgacagtagttcttccttctctccagcaagttttcgtagccttacatctaatggcccttctcctgctgactccaagacctgagcagcttcctgagacacaacagtgatggctccagccactggttcatgactgacatcaccattgggagtgccatcggggattataactaagccatgtttctcaataagctcatctctttgccgcaggccttctttaagttcttccatcttatgctgcagcacactacacatatgtttctgcctttctaactcctttgatttttcttcattttctctataaaattctgccatctgttcctcctgctcttcaataacatccttgagtgtgtctacttggtagatcaaattgttcttctcattgtctaactgtgcattggaaaccatggctttcttgtatttttcttccacttcagacaaagattcccgcaattcacttaatgaagtgtctggatctattaagctgctggtgtccccacttcctcgtctggatgagtttccacttagaggggttgttgctgaggcagaatttcgagatgaaggtcttgtataattttcagcatactgtttgtcagatttttcatccaactctttttgttgtcgttccagttctctcatgcgtatatctcttgcttctgcccgggcagcccgttttgctgccagccttgcctctgcctctctggcaatgttactcaaagcttcatcttctgcagaaaatcggtctttcacaggtgttcttttccttccagaagcaggagtccccatcttgtgttcttaatagtcttttaactttgaaagtgatttaactgtgttttcagcccttagtgatggtagctctcctttccactgacatttacatctagaccccttcatttatcttcccacatctgtgttagggcgcgcgctgcgactgcgtcgctgtccgggaagggccgaagagctgctcgcccgcccggcgcccgctggggctatgggcgaggggcgcagctggacgactcagtcctgggtccccggccaggcgggcggggatggacgcggcggctcccggcactggcagccggctagtcggtcaggccgatgtgccctctgcgccgcggctgagacagcgggaaccggccccgggaggagccgcagcctgagcggccgactgaggaggcgaaggatgggcggggccacagggtcgacgac

SEQ ID NO: 16380 - RNA, 2671 nt, Homo sapiens
  source 1..2671: mol_type = other RNA
gtccacttctgcctgccctgccctaccctccccctttgggtttgtttgaggtttcattccacaaataagcagcagataaaatactttacaaggtacagcacagttgtattgaagaaaaaaaggacccaactcttactttaggagtattaggcctggacttcccctgccccatgcaataaagcaagttttatatacactccccatatttttttctaacattttcttatataaatttaaatattttacaaaaaaaggcttttttcctccaaacatataaatctgagtgaaacatagattccccacccgagaacttgtttcttcactaaaatataaatgttgtctgatattaagggtaaatgtcttttgaccactggagatcactgaagtctgaattgcaccgtggagaaggcacttgtgttttctgaggtctccagcaagtatctcagtgagcactcatagaattgctgtctgtcctccagaacccgtgccaaggcctccgagtgcccagttactgaggcagctggggaaaaacgttgagtaaacatgattctacaattacggagataaaaaataaaaacagcatggactggttctaccctagaatcaaactacaacaaaatccaaagtgttcattcatgtagattcaaaatgacttcattctgtcataaattataaaatacaaaggtggctgttttaatgacaaaactcaaaacagtactaaaaggggtttgtgtcaatggacaaaagtcagtccctctaggtagggccccaaggagcatcacccaggttgaagggtggttttcctactgctgggccagaagtgctgtcctattggccttcatcttctccagccgcttggccaggtggctgttggtcatctccatctcctcaatcttgtccagtgctgttcgtaactctcgttgtagcttccgtttttctgctttcaattcatcttcaactttctcagcattctcagcagcagttttatatctcagaacctgtccctcaagccggctaatactttgctccaaggtagttatatcctgttctgcttttgaaagcttaaatttgtattcgctaatttgtctattggcatctctctgcatttcgatgaactgcaagtctgagccattctgcagtcctgccaggtcacccactgtgccatcattcctggagcatttctgtcgttcctcctctaactgaagcttcagttttctaatctgtgacagtagttcttccttctctccagcaagttttcgtagccttacatctaatggcccttctcctgctgactccaagacctgagcagcttcctgagacacaacagtgatggctccagccactggttcatgactgacatcaccattgggagtgccatcggggattataactaagccatgtttctcaataagctcatctctttgccgcaggccttctttaagttcttccatcttatgctgcagcacactacacatatgtttctgcctttctaactcctttgatttttcttcattttctctataaaattctgccatctgttcctcctgctcttcaataacatccttgagtgtgtctacttggtagatcaaattgttcttctcattgtctaactgtgcattggaaaccatggctttcttgtatttttcttccacttcagacaaagattcccgcaattcacttaatgaagtgtctggatctattaagctgctggtgtccccacttcctcgtctggatgagtttccacttagaggggttgttgctgaggcagaatttcgagatgaaggtcttgtataattttcagcatactgtttgtcagatttttcatccaactctttttgttgtcgttccagttctctcatgcgtatatctcttgcttctgcccgggcagcccgttttgctgccagccttgcctctgcctctctggcaatgttactcaaagcttcatcttctgcagaaaatcggtctttcacaggtgttcttttccttccagaagcaggagtccccatcttgtgttcttaatagtcttttaactttgaaagtgatttaactgtgttttcagcccttagtgatggtagctctcctttccactgacatttacatctagaccccttcatttatcttcccacatcttttccccagcgcggtggaagggtgagcgttagaaatcagacgggatgtctgagaacgccgcaggcagggggcgaccccagcccgggagcccgccgcgggccggccagtccccagggaagcccggccccctagccgaggtcggaggcggcgcggatcccacgggactgcggaggccgggaaaaaggttcccaactccccgctccctgctcccaccgggctggcgggaggagcggcccttacctgtgttagggcgcgcgctgcgactgcgtcgctgtccgggaagggccgaagagctgctcgcccgcccggcgcccgctggggctatgggcgaggggcgcagctggacgactcagtcctgggtccccggccaggcgggcggggatggacgcggcggctcccggcactggcagccggctagtcggtcaggccgatgtgccctctgcgccgcggctgagacagcgggaaccggccccgggaggagccgcagcctgagcggccgactgaggaggcgaaggatgggcggggccacagggtcgacgac

SEQ ID NO: 16381 - RNA, 3092 nt, Homo sapiens
  source 1..3092: mol_type = other RNA
gtccacttctgcctgccctgccctaccctccccctttgggtttgtttgaggtttcattccacaaataagcagcagataaaatactttacaaggtacagcacagttgtattgaagaaaaaaaggacccaactcttactttaggagtattaggcctggacttcccctgccccatgcaataaagcaagttttatatacactccccatatttttttctaacattttcttatataaatttaaatattttacaaaaaaaggcttttttcctccaaacatataaatctgagtgaaacatagattccccacccgagaacttgtttcttcactaaaatataaatgttgtctgatattaagggtaaatgtcttttgaccactggagatcactgaagtctgaattgcaccgtggagaaggcacttgtgttttctgaggtctccagcaagtatctcagtgagcactcatagaattgctgtctgtcctccagaacccgtgccaaggcctccgagtgcccagttactgaggcagctggggaaaaacgttgagtaaacatgattctacaattacggagataaaaaataaaaacagcatggactggttctaccctagaatcaaactacaacaaaatccaaagtgttcattcatgtagattcaaaatgacttcattctgtcataaattataaaatacaaaggtggctgttttaatgacaaaactcaaaacagtactaaaaggggtttgtgtcaatggacaaaagtcagtccctctaggtagggccccaaggagcatcacccaggttgaagggtggttttcctactgctgggccagaagtgctgtcctattggccttcatcttctccagccgcttggccaggtggctgttggtcatctccatctcctcaatcttgtccagtgctgttcgtaactctcgttgtagcttccgtttttctgctttcaattcatcttcaactttctcagcattctcagcagcagttttatatctcagaacctgtccctcaagccggctaatactttgctccaaggtagttatatcctgttctgcttttgaaagcttaaatttgtattcgctaatttgtctattggcatctctctgcatttcgatgaactgcaagtctgagccattctgcagtcctgccaggtcacccactgtgccatcattcctggagcatttctgtcgttcctcctctaactgaagcttcagttttctaatctgtgacagtagttcttccttctctccagcaagttttcgtagccttacatctaatggcccttctcctgctgactccaagacctgagcagcttcctgagacacaacagtgatggctccagccactggttcatgactgacatcaccattgggagtgccatcggggattataactaagccatgtttctcaataagctcatctctttgccgcaggccttctttaagttcttccatcttatgctgcagcacactacacatatgtttctgcctttctaactcctttgatttttcttcattttctctataaaattctgccatctgttcctcctgctcttcaataacatccttgagtgtgtctacttggtagatcaaattgttcttctcattgtctaactgtgcattggaaaccatggctttcttgtatttttcttccacttcagacaaagattcccgcaattcacttaatgaagtgtctggatctattaagctgctggtgtccccacttcctcgtctggatgagtttccacttagaggggttgttgctgaggcagaatttcgagatgaaggtcttgtataattttcagcatactgtttgtcagatttttcatccaagctggacaaatctgggatactgatatcatccacctcagagacaacacttcccctacgattggagcgactgaaataatcagcggcagataccacactctcccttcgtccacgactggcacgatcagaagacacaatgcttgcagtgtcatcgttggtaaaccctggactgcttcgggctgaacttattcttgatgaataataactgcattcagatggagttcgaggaccataagggttatataatccaccattgtacaatgatgccagactggcacttctcagcagaccagaatttgcagtaggagaggccctgtcactcttatatgttgccagagggtcactgtacagggaagaagactgccgagtgtagtaggcagaggtgggtttgctatgtctaagactgctatagtttctctggtcaaagtagaggccactcagtaggtctttatgagaatcagaagacctcttcttcattccatgagagtgactgtaagaatgatttaatgatgaaagtcttgatgatctatccttgaacatatcatacctgtgactgccaacacttcgaatggacaatgcatcctcaactcccagataaggacgatggtgactggaccggtgggaatacctggccctttccgaatcttccagccacttctgaatctgtccccacttccgatcaaaggaatgaagagagtactctttttgttgtcgttccagttctctcatgcgtatatctcttgcttctgcccgggcagcccgttttgctgccagccttgcctctgcctctctggcaatgttactcaaagcttcatcttctgcagaaaatcggtctttcacaggtgttcttttccttccagaagcaggagtccccatcttgtgttcttaatagtcttttaactttgaaagtgatttaactgtgttttcagcccttagtgatggtagctctcctttccactgacatttacatctagaccccttcatttatcttcccacatctgtgttagggcgcgcgctgcgactgcgtcgctgtccgggaagggccgaagagctgctcgcccgcccggcgcccgctggggctatgggcgaggggcgcagctggacgactcagtcctgggtccccggccaggcgggcggggatggacgcggcggctcccggcactggcagccggctagtcggtcaggccgatgtgccctctgcgccgcggctgagacagcgggaaccggccccgggaggagccgcagcctgagcggccgactgaggag

SEQ ID NO: 16382 - RNA, 2570 nt, Homo sapiens
  source 1..2570: mol_type = other RNA
gtccacttctgcctgccctgccctaccctccccctttgggtttgtttgaggtttcattccacaaataagcagcagataaaatactttacaaggtacagcacagttgtattgaagaaaaaaaggacccaactcttactttaggagtattaggcctggacttcccctgccccatgcaataaagcaagttttatatacactccccatatttttttctaacattttcttatataaatttaaatattttacaaaaaaaggcttttttcctccaaacatataaatctgagtgaaacatagattccccacccgagaacttgtttcttcactaaaatataaatgttgtctgatattaagggtaaatgtcttttgaccactggagatcactgaagtctgaattgcaccgtggagaaggcacttgtgttttctgaggtctccagcaagtatctcagtgagcactcatagaattgctgtctgtcctccagaacccgtgccaaggcctccgagtgcccagttactgaggcagctggggaaaaacgttgagtaaacatgattctacaattacggagataaaaaataaaaacagcatggactggttctaccctagaatcaaactacaacaaaatccaaagtgttcattcatgtagattcaaaatgacttcattctgtcataaattataaaatacaaaggtggctgttttaatgacaaaactcaaaacagtactaaaaggggtttgtgtcaatggacaaaagtcagtccctctaggtagggccccaaggagcatcacccaggttgaagggtggttttcctactgctgggccagaagtgctgtcctattggccttcatcttctccagccgcttggccaggtggctgttggtcatctccatctcctcaatcttgtccagtgctgttcgtaactctcgttgtagcttccgtttttctgctttcaattcatcttcaactttctcagcattctcagcagcagttttatatctcagaacctgtccctcaagccggctaatactttgctccaaggtagttatatcctgttctgcttttgaaagcttaaatttgtattcgctaatttgtctattggcatctctctgcatttcgatgaactgcaagtctgagccattctgcagtcctgccaggtcacccactgtgccatcattcctggagcatttctgtcgttcctcctctaactgaagcttcagttttctaatctgtgacagtagttcttccttctctccagcaagttttcgtagccttacatctaatggcccttctcctgctgactccaagacctgagcagcttcctgagacacaacagtgatggctccagccactggttcatgactgacatcaccattgggagtgccatcggggattataactaagccatgtttctcaataagctcatctctttgccgcaggccttctttaagttcttccatcttatgctgcagcacactacacatatgtttctgcctttctaactcctttgatttttcttcattttctctataaaattctgccatctgttcctcctgctcttcaataacatccttgagtgtgtctacttggtagatcaaattgttcttctcattgtctaactgtgcattggaaaccatggctttcttgtatttttcttccacttcagacaaagattcctttagttctttaagcccctgcatgtatctcccttctacatcctgtatctggtccttaaggtcatagatatcccgcaattcacttaatgaagtgtctggatctattaagctgctggtgtccccacttcctcgtctggatgagtttccacttagaggggttgttgctgaggcagaatttcgagatgaaggtcttgtataattttcagcatactgtttgtcagatttttcatccaacctgtgactgccaacacttcgaatggacaatgcatcctcaactcccagataaggacgatggtgactggaccggtgggaatacctggccctttccgaatcttcctctttttgttgtcgttccagttctctcatgcgtatatctcttgcttctgcccgggcagcccgttttgctgccagccttgcctctgcctctctggcaatgttactcaaagcttcatcttctgcagaaaatcggtctttcacaggtgttcttttccttccagaagcaggagtccccatcttgtgttcttaatagtcttttaactttgaaagtgatttaactgtgttttcagcccttagtgatggtagctctcctttccactgacatttacatctagaccccttcatttatcttcccacatctgtgttagggcgcgcgctgcgactgcgtcgctgtccgggaagggccgaagagctgctcgcccgcccggcgcccgctggggctatgggcgaggggcgcagctggacgactcagtcctgggtccccggccaggcgggcggggatggacgcggcggctcccggcactggcagccggctagtcggtcaggccgatgtgccctctgcgccgcggctgagacagcgggaaccggccccgggaggagccgcagcctgagcggccgactgaggag

SEQ ID NO: 16383 - RNA, 2511 nt, Homo sapiens
  source 1..2511: mol_type = other RNA
gtccacttctgcctgccctgccctaccctccccctttgggtttgtttgaggtttcattccacaaataagcagcagataaaatactttacaaggtacagcacagttgtattgaagaaaaaaaggacccaactcttactttaggagtattaggcctggacttcccctgccccatgcaataaagcaagttttatatacactccccatatttttttctaacattttcttatataaatttaaatattttacaaaaaaaggcttttttcctccaaacatataaatctgagtgaaacatagattccccacccgagaacttgtttcttcactaaaatataaatgttgtctgatattaagggtaaatgtcttttgaccactggagatcactgaagtctgaattgcaccgtggagaaggcacttgtgttttctgaggtctccagcaagtatctcagtgagcactcatagaattgctgtctgtcctccagaacccgtgccaaggcctccgagtgcccagttactgaggcagctggggaaaaacgttgagtaaacatgattctacaattacggagataaaaaataaaaacagcatggactggttctaccctagaatcaaactacaacaaaatccaaagtgttcattcatgtagattcaaaatgacttcattctgtcataaattataaaatacaaaggtggctgttttaatgacaaaactcaaaacagtactaaaaggggtttgtgtcaatggacaaaagtcagtccctctaggtagggccccaaggagcatcacccaggttgaagggtggttttcctactgctgggccagaagtgctgtcctattggccttcatcttctccagccgcttggccaggtggctgttggtcatctccatctcctcaatcttgtccagtgctgttcgtaactctcgttgtagcttccgtttttctgctttcaattcatcttcaactttctcagcattctcagcagcagttttatatctcagaacctgtccctcaagccggctaatactttgctccaaggtagttatatcctgttctgcttttgaaagcttaaatttgtattcgctaatttgtctattggcatctctctgcatttcgatgaactgcaagtctgagccattctgcagtcctgccaggtcacccactgtgccatcattcctggagcatttctgtcgttcctcctctaactgaagcttcagttttctaatctgtgacagtagttcttccttctctccagcaagttttcgtagccttacatctaatggcccttctcctgctgactccaagacctgagcagcttcctgagacacaacagtgatggctccagccactggttcatgactgacatcaccattgggagtgccatcggggattataactaagccatgtttctcaataagctcatctctttgccgcaggccttctttaagttcttccatcttatgctgcagcacactacacatatgtttctgcctttctaactcctttgatttttcttcattttctctataaaattctgccatctgttcctcctgctcttcaataacatccttgagtgtgtctacttggtagatcaaattgttcttctcattgtctaactgtgcattggaaaccatggctttcttgtatttttcttccacttcagacaaagattcctttagttctttaagcccctgcatgtatctcccttctacatcctgtatctggtccttaaggtcatagatatcccgcaattcacttaatgaagtgtctggatctattaagctgctggtgtccccacttcctcgtctggatgagtttccacttagaggggttgttgctgaggcagaatttcgagatgaaggtcttgtataattttcagcatactgtttgtcagatttttcatccaactctttttgttgtcgttccagttctctcatgcgtatatctcttgcttctgcccgggcagcccgttttgctgccagccttgcctctgcctctctggcaatgttactcaaagcttcatcttctgcagaaaatcggtctttcacaggtgttcttttccttccagaagcaggagtccccatcttgtgttcttaatagtcttttaactttgaaagtgatttaactgtgttttcagccagaaaagaaggaaagtatcttcaggatcttgcagaatataaaccttagtgatggtagctctcctttccactgacatttacatctagaccccttcatttatcttcccacatctgtgttagggcgcgcgctgcgactgcgtcgctgtccgggaagggccgaagagctgctcgcccgcccggcgcccgctggggctatgggcgaggggcgcagctggacgactcagtcctgggtccccggccaggcgggcggggatggacgcggcggctcccggcactggcagccggctagtcggtcaggccgatgtgccctctgcgccgcggctgagacagcgggaaccggccccgggaggagccgcagcctgagcggccgactgaggag

SEQ ID NO: 16384 - RNA, 2501 nt, Homo sapiens
  source 1..2501: mol_type = other RNA
gtccacttctgcctgccctgccctaccctccccctttgggtttgtttgaggtttcattccacaaataagcagcagataaaatactttacaaggtacagcacagttgtattgaagaaaaaaaggacccaactcttactttaggagtattaggcctggacttcccctgccccatgcaataaagcaagttttatatacactccccatatttttttctaacattttcttatataaatttaaatattttacaaaaaaaggcttttttcctccaaacatataaatctgagtgaaacatagattccccacccgagaacttgtttcttcactaaaatataaatgttgtctgatattaagggtaaatgtcttttgaccactggagatcactgaagtctgaattgcaccgtggagaaggcacttgtgttttctgaggtctccagcaagtatctcagtgagcactcatagaattgctgtctgtcctccagaacccgtgccaaggcctccgagtgcccagttactgaggcagctggggaaaaacgttgagtaaacatgattctacaattacggagataaaaaataaaaacagcatggactggttctaccctagaatcaaactacaacaaaatccaaagtgttcattcatgtagattcaaaatgacttcattctgtcataaattataaaatacaaaggtggctgttttaatgacaaaactcaaaacagtactaaaaggggtttgtgtcaatggacaaaagtcagtccctctaggtagggccccaaggagcatcacccaggttgaagggtggttttcctactgctgggccagaagtgctgtcctattggccttcatcttctccagccgcttggccaggtggctgttggtcatctccatctcctcaatcttgtccagtgctgttcgtaactctcgttgtagcttccgtttttctgctttcaattcatcttcaactttctcagcattctcagcagcagttttatatctcagaacctgtccctcaagccggctaatactttgctccaaggtagttatatcctgttctgcttttgaaagcttaaatttgtattcgctaatttgtctattggcatctctctgcatttcgatgaactgcaagtctgagccattctgcagtcctgccaggtcacccactgtgccatcattcctggagcatttctgtcgttcctcctctaactgaagcttcagttttctaatctgtgacagtagttcttccttctctccagcaagttttcgtagccttacatctaatggcccttctcctgctgactccaagacctgagcagcttcctgagacacaacagtgatggctccagccactggttcatgactgacatcaccattgggagtgccatcggggattataactaagccatgtttctcaataagctcatctctttgccgcaggccttctttaagttcttccatcttatgctgcagcacactacacatatgtttctgcctttctaactcctttgatttttcttcattttctctataaaattctgccatctgttcctcctgctcttcaataacatccttgagtgtgtctacttggtagatcaaattgttcttctcattgtctaactgtgcattggaaaccatggctttcttgtatttttcttccacttcagacaaagattcctttagttctttaagcccctgcatgtatctcccttctacatcctgtatctggtccttaaggtcatagatatcccgcaattcacttaatgaagtgtctggatctattaagctgctggtgtccccacttcctcgtctggatgagtttccacttagaggggttgttgctgaggcagaatttcgagatgaaggtcttgtataattttcagcatactgtttgtcagatttttcatccaactctttttgttgtcgttccagttctctcatgcgtatatctcttgcttctgcccgggcagcccgttttgctgccagccttgcctctgcctctctggcaatgttactcaaagcttcatcttctgcagaaaatcggtctttcacaggtgttcttttccttccagaagcaggagtccccatcttgtgttcttaatagtcttttaactttgaaagtgatttaactgtgttttcagcccttagtgatggtagctctcctttccactgacatttacatctagaccccttcatttatcttcccacatctgtgttagggcgcgcgctgcgactgcgtcgctgtccgggaagggccgaagagctgctcgcccgcccggcgcccgctggggctatgggcgaggggcgcagctggacgactcagtcctgggtccccggccaggcgggcggggatggacgcggcggctcccggcactggcagccggctagtcggtcaggccgatgtgccctctgcgccgcggctgagacagcgggaaccggccccgggaggagccgcagcctgagcggccgactgaggaggcgaaggatgggcggggccacagggtcgacgac

SEQ ID NO: 16385 - RNA, 2743 nt, Homo sapiens
  source 1..2743: mol_type = other RNA
gtccacttctgcctgccctgccctaccctccccctttgggtttgtttgaggtttcattccacaaataagcagcagataaaatactttacaaggtacagcacagttgtattgaagaaaaaaaggacccaactcttactttaggagtattaggcctggacttcccctgccccatgcaataaagcaagttttatatacactccccatatttttttctaacattttcttatataaatttaaatattttacaaaaaaaggcttttttcctccaaacatataaatctgagtgaaacatagattccccacccgagaacttgtttcttcactaaaatataaatgttgtctgatattaagggtaaatgtcttttgaccactggagatcactgaagtctgaattgcaccgtggagaaggcacttgtgttttctgaggtctccagcaagtatctcagtgagcactcatagaattgctgtctgtcctccagaacccgtgccaaggcctccgagtgcccagttactgaggcagctggggaaaaacgttgagtaaacatgattctacaattacggagataaaaaataaaaacagcatggactggttctaccctagaatcaaactacaacaaaatccaaagtgttcattcatgtagattcaaaatgacttcattctgtcataaattataaaatacaaaggtggctgttttaatgacaaaactcaaaacagtactaaaaggggtttgtgtcaatggacaaaagtcagtccctctaggtagggccccaaggagcatcacccaggttgaagggtggttttcctactgctgggccagaagtgctgtcctattggccttcatcttctccagccgcttggccaggtggctgttggtcatctccatctcctcaatcttgtccagtgctgttcgtaactctcgttgtagcttccgtttttctgctttcaattcatcttcaactttctcagcattctcagcagcagttttatatctcagaacctgtccctcaagccggctaatactttgctccaaggtagttatatcctgttctgcttttgaaagcttaaatttgtattcgctaatttgtctattggcatctctctgcatttcgatgaactgcaagtctgagccattctgcagtcctgccaggtcacccactgtgccatcattcctggagcatttctgtcgttcctcctctaactgaagcttcagttttctaatctgtgacagtagttcttccttctctccagcaagttttcgtagccttacatctaatggcccttctcctgctgactccaagacctgagcagcttcctgagacacaacagtgatggctccagccactggttcatgactgacatcaccattgggagtgccatcggggattataactaagccatgtttctcaataagctcatctctttgccgcaggccttctttaagttcttccatcttatgctgcagcacactacacatatgtttctgcctttctaactcctttgatttttcttcattttctctataaaattctgccatctgttcctcctgctcttcaataacatccttgagtgtgtctacttggtagatcaaattgttcttctcattgtctaactgtgcattggaaaccatggctttcttgtatttttcttccacttcagacaaagattcctttagttctttaagcccctgcatgtatctcccttctacatcctgtatctggtccttaaggtcatagatatcccgcaattcacttaatgaagtgtctggatctattaagctgctggtgtccccacttcctcgtctggatgagtttccacttagaggggttgttgctgaggcagaatttcgagatgaaggtcttgtataattttcagcatactgtttgtcagatttttcatccaactctttttgttgtcgttccagttctctcatgcgtatatctcttgcttctgcccgggcagcccgttttgctgccagccttgcctctgcctctctggcaatgttactcaaagcttcatcttctgcagaaaatcggtctttcacaggtgttcttttccttccagaagcaggagtccccatcttgtgttcttaatagtcttttaactttgaaagtgatttaactgtgttttcagcccttagtgatggtagctctcctttccactgacatttacatctagaccccttcatttatcttcccacatcttttccccagcgcggtggaagggtgagcgttagaaatcagacgggatgtctgagaacgccgcaggcagggggcgaccccagcccgggagcccgccgcgggccggccagtccccagggaagcccggccccctagccgaggtcggaggcggcgcggatcccacgggactgcggaggccgggaaaaaggttcccaactccccgctccctgctcccaccgggctggcgggaggagcggcccttacctgtgttagggcgcgcgctgcgactgcgtcgctgtccgggaagggccgaagagctgctcgcccgcccggcgcccgctggggctatgggcgaggggcgcagctggacgactcagtcctgggtccccggccaggcgggcggggatggacgcggcggctcccggcactggcagccggctagtcggtcaggccgatgtgccctctgcgccgcggctgagacagcgggaaccggccccgggaggagccgcagcctgagcggccgactgaggaggcgaaggatgggcggggccacagggtcgacgac

SEQ ID NO: 16386 - RNA, 3164 nt, Homo sapiens
  source 1..3164: mol_type = other RNA
gtccacttctgcctgccctgccctaccctccccctttgggtttgtttgaggtttcattccacaaataagcagcagataaaatactttacaaggtacagcacagttgtattgaagaaaaaaaggacccaactcttactttaggagtattaggcctggacttcccctgccccatgcaataaagcaagttttatatacactccccatatttttttctaacattttcttatataaatttaaatattttacaaaaaaaggcttttttcctccaaacatataaatctgagtgaaacatagattccccacccgagaacttgtttcttcactaaaatataaatgttgtctgatattaagggtaaatgtcttttgaccactggagatcactgaagtctgaattgcaccgtggagaaggcacttgtgttttctgaggtctccagcaagtatctcagtgagcactcatagaattgctgtctgtcctccagaacccgtgccaaggcctccgagtgcccagttactgaggcagctggggaaaaacgttgagtaaacatgattctacaattacggagataaaaaataaaaacagcatggactggttctaccctagaatcaaactacaacaaaatccaaagtgttcattcatgtagattcaaaatgacttcattctgtcataaattataaaatacaaaggtggctgttttaatgacaaaactcaaaacagtactaaaaggggtttgtgtcaatggacaaaagtcagtccctctaggtagggccccaaggagcatcacccaggttgaagggtggttttcctactgctgggccagaagtgctgtcctattggccttcatcttctccagccgcttggccaggtggctgttggtcatctccatctcctcaatcttgtccagtgctgttcgtaactctcgttgtagcttccgtttttctgctttcaattcatcttcaactttctcagcattctcagcagcagttttatatctcagaacctgtccctcaagccggctaatactttgctccaaggtagttatatcctgttctgcttttgaaagcttaaatttgtattcgctaatttgtctattggcatctctctgcatttcgatgaactgcaagtctgagccattctgcagtcctgccaggtcacccactgtgccatcattcctggagcatttctgtcgttcctcctctaactgaagcttcagttttctaatctgtgacagtagttcttccttctctccagcaagttttcgtagccttacatctaatggcccttctcctgctgactccaagacctgagcagcttcctgagacacaacagtgatggctccagccactggttcatgactgacatcaccattgggagtgccatcggggattataactaagccatgtttctcaataagctcatctctttgccgcaggccttctttaagttcttccatcttatgctgcagcacactacacatatgtttctgcctttctaactcctttgatttttcttcattttctctataaaattctgccatctgttcctcctgctcttcaataacatccttgagtgtgtctacttggtagatcaaattgttcttctcattgtctaactgtgcattggaaaccatggctttcttgtatttttcttccacttcagacaaagattcctttagttctttaagcccctgcatgtatctcccttctacatcctgtatctggtccttaaggtcatagatatcccgcaattcacttaatgaagtgtctggatctattaagctgctggtgtccccacttcctcgtctggatgagtttccacttagaggggttgttgctgaggcagaatttcgagatgaaggtcttgtataattttcagcatactgtttgtcagatttttcatccaagctggacaaatctgggatactgatatcatccacctcagagacaacacttcccctacgattggagcgactgaaataatcagcggcagataccacactctcccttcgtccacgactggcacgatcagaagacacaatgcttgcagtgtcatcgttggtaaaccctggactgcttcgggctgaacttattcttgatgaataataactgcattcagatggagttcgaggaccataagggttatataatccaccattgtacaatgatgccagactggcacttctcagcagaccagaatttgcagtaggagaggccctgtcactcttatatgttgccagagggtcactgtacagggaagaagactgccgagtgtagtaggcagaggtgggtttgctatgtctaagactgctatagtttctctggtcaaagtagaggccactcagtaggtctttatgagaatcagaagacctcttcttcattccatgagagtgactgtaagaatgatttaatgatgaaagtcttgatgatctatccttgaacatatcatacctgtgactgccaacacttcgaatggacaatgcatcctcaactcccagataaggacgatggtgactggaccggtgggaatacctggccctttccgaatcttccagccacttctgaatctgtccccacttccgatcaaaggaatgaagagagtactctttttgttgtcgttccagttctctcatgcgtatatctcttgcttctgcccgggcagcccgttttgctgccagccttgcctctgcctctctggcaatgttactcaaagcttcatcttctgcagaaaatcggtctttcacaggtgttcttttccttccagaagcaggagtccccatcttgtgttcttaatagtcttttaactttgaaagtgatttaactgtgttttcagcccttagtgatggtagctctcctttccactgacatttacatctagaccccttcatttatcttcccacatctgtgttagggcgcgcgctgcgactgcgtcgctgtccgggaagggccgaagagctgctcgcccgcccggcgcccgctggggctatgggcgaggggcgcagctggacgactcagtcctgggtccccggccaggcgggcggggatggacgcggcggctcccggcactggcagccggctagtcggtcaggccgatgtgccctctgcgccgcggctgagacagcgggaaccggccccgggaggagccgcagcctgagcggccgactgaggag

SEQ ID NO: 16387 - RNA, 2693 nt, Homo sapiens
  source 1..2693: mol_type = other RNA
gtccacttctgcctgccctgccctaccctccccctttgggtttgtttgaggtttcattccacaaataagcagcagataaaatactttacaaggtacagcacagttgtattgaagaaaaaaaggacccaactcttactttaggagtattaggcctggacttcccctgccccatgcaataaagcaagttttatatacactccccatatttttttctaacattttcttatataaatttaaatattttacaaaaaaaggcttttttcctccaaacatataaatctgagtgaaacatagattccccacccgagaacttgtttcttcactaaaatataaatgttgtctgatattaagggtaaatgtcttttgaccactggagatcactgaagtctgaattgcaccgtggagaaggcacttgtgttttctgaggtctccagcaagtatctcagtgagcactcatagaattgctgtctgtcctccagaacccgtgccaaggcctccgagtgcccagttactgaggcagctggggaaaaacgttgagtaaacatgattctacaattacggagataaaaaataaaaacagcatggactggttctaccctagaatcaaactacaacaaaatccaaagtgttcattcatgtagattcaaaatgacttcattctgtcataaattataaaatacaaaggtggctgttttaatgacaaaactcaaaacagtactaaaaggggtttgtgtcaatggacaaaagtcagtccctctaggtagggccccaaggagcatcacccaggttgaagggtggttttcctactgctgggccagaagtgctgtcctattggccttcatcttctccagccgcttggccaggtggctgttggtcatctccatctcctcaatcttgtccagtgctgttcgtaactctcgttgtagcttccgtttttctgctttcaattcatcttcaactttctcagcattctcagcagcagttttatatctcagaacctgtccctcaagccggctaatactttgctccaaggtagttatatcctgttctgcttttgaaagcttaaatttgtattcgctaatttgtctattggcatctctctgcatttcgatgaactgcaagtctgagccattctgcagtcctgccaggtcacccactgtgccatcattcctggagcatttctgtcgttcctcctctaactgaagcttcagttttctaatctgtgacagtagttcttccttctctccagcaagttttcgtagccttacatctaatggcccttctcctgctgactccaagacctgagcagcttcctgagacacaacagtgatggctccagccactggttcatgactgacatcaccattgggagtgccatcggggattataactaagccatgtttctctcccgtcttcactgtctcctgcaggtcagccagctcctctctgagcatatctcgctcattcctaaggcaggcaatgtattctttctgtttctctagggccccaatttttttatctttccaaagaagtgtctcctggaggtcaaacacctcttttgtcatggtgtctattttctgctgcatgcgctgcttctcctcaataagctcatctctttgccgcaggccttctttaagttcttccatcttatgctgcagcacactacacatatgtttctgcctttctaactcctttgatttttcttcattttctctataaaattctgccatctgttcctcctgctcttcaataacatccttgagtgtgtctacttggtagatcaaattgttcttctcattgtctaactgtgcattggaaaccatggctttcttgtatttttcttccacttcagacaaagattcccgcaattcacttaatgaagtgtctggatctattaagctgctggtgtccccacttcctcgtctggatgagtttccacttagaggggttgttgctgaggcagaatttcgagatgaaggtcttgtataattttcagcatactgtttgtcagatttttcatccaacctgtgactgccaacacttcgaatggacaatgcatcctcaactcccagataaggacgatggtgactggaccggtgggaatacctggccctttccgaatcttcctctttttgttgtcgttccagttctctcatgcgtatatctcttgcttctgcccgggcagcccgttttgctgccagccttgcctctgcctctctggcaatgttactcaaagcttcatcttctgcagaaaatcggtctttcacaggtgttcttttccttccagaagcaggagtccccatcttgtgttcttaatagtcttttaactttgaaagtgatttaactgtgttttcagcccttagtgatggtagctctcctttccactgacatttacatctagaccccttcatttatcttcccacatctgtgttagggcgcgcgctgcgactgcgtcgctgtccgggaagggccgaagagctgctcgcccgcccggcgcccgctggggctatgggcgaggggcgcagctggacgactcagtcctgggtccccggccaggcgggcggggatggacgcggcggctcccggcactggcagccggctagtcggtcaggccgatgtgccctctgcgccgcggctgagacagcgggaaccggccccgggaggagccgcagcctgagcggccgactgaggag

SEQ ID NO: 16388 - RNA, 2624 nt, Homo sapiens
  source 1..2624: mol_type = other RNA
gtccacttctgcctgccctgccctaccctccccctttgggtttgtttgaggtttcattccacaaataagcagcagataaaatactttacaaggtacagcacagttgtattgaagaaaaaaaggacccaactcttactttaggagtattaggcctggacttcccctgccccatgcaataaagcaagttttatatacactccccatatttttttctaacattttcttatataaatttaaatattttacaaaaaaaggcttttttcctccaaacatataaatctgagtgaaacatagattccccacccgagaacttgtttcttcactaaaatataaatgttgtctgatattaagggtaaatgtcttttgaccactggagatcactgaagtctgaattgcaccgtggagaaggcacttgtgttttctgaggtctccagcaagtatctcagtgagcactcatagaattgctgtctgtcctccagaacccgtgccaaggcctccgagtgcccagttactgaggcagctggggaaaaacgttgagtaaacatgattctacaattacggagataaaaaataaaaacagcatggactggttctaccctagaatcaaactacaacaaaatccaaagtgttcattcatgtagattcaaaatgacttcattctgtcataaattataaaatacaaaggtggctgttttaatgacaaaactcaaaacagtactaaaaggggtttgtgtcaatggacaaaagtcagtccctctaggtagggccccaaggagcatcacccaggttgaagggtggttttcctactgctgggccagaagtgctgtcctattggccttcatcttctccagccgcttggccaggtggctgttggtcatctccatctcctcaatcttgtccagtgctgttcgtaactctcgttgtagcttccgtttttctgctttcaattcatcttcaactttctcagcattctcagcagcagttttatatctcagaacctgtccctcaagccggctaatactttgctccaaggtagttatatcctgttctgcttttgaaagcttaaatttgtattcgctaatttgtctattggcatctctctgcatttcgatgaactgcaagtctgagccattctgcagtcctgccaggtcacccactgtgccatcattcctggagcatttctgtcgttcctcctctaactgaagcttcagttttctaatctgtgacagtagttcttccttctctccagcaagttttcgtagccttacatctaatggcccttctcctgctgactccaagacctgagcagcttcctgagacacaacagtgatggctccagccactggttcatgactgacatcaccattgggagtgccatcggggattataactaagccatgtttctctcccgtcttcactgtctcctgcaggtcagccagctcctctctgagcatatctcgctcattcctaaggcaggcaatgtattctttctgtttctctagggccccaatttttttatctttccaaagaagtgtctcctggaggtcaaacacctcttttgtcatggtgtctattttctgctgcatgcgctgcttctcctcaataagctcatctctttgccgcaggccttctttaagttcttccatcttatgctgcagcacactacacatatgtttctgcctttctaactcctttgatttttcttcattttctctataaaattctgccatctgttcctcctgctcttcaataacatccttgagtgtgtctacttggtagatcaaattgttcttctcattgtctaactgtgcattggaaaccatggctttcttgtatttttcttccacttcagacaaagattcccgcaattcacttaatgaagtgtctggatctattaagctgctggtgtccccacttcctcgtctggatgagtttccacttagaggggttgttgctgaggcagaatttcgagatgaaggtcttgtataattttcagcatactgtttgtcagatttttcatccaactctttttgttgtcgttccagttctctcatgcgtatatctcttgcttctgcccgggcagcccgttttgctgccagccttgcctctgcctctctggcaatgttactcaaagcttcatcttctgcagaaaatcggtctttcacaggtgttcttttccttccagaagcaggagtccccatcttgtgttcttaatagtcttttaactttgaaagtgatttaactgtgttttcagcccttagtgatggtagctctcctttccactgacatttacatctagaccccttcatttatcttcccacatctgtgttagggcgcgcgctgcgactgcgtcgctgtccgggaagggccgaagagctgctcgcccgcccggcgcccgctggggctatgggcgaggggcgcagctggacgactcagtcctgggtccccggccaggcgggcggggatggacgcggcggctcccggcactggcagccggctagtcggtcaggccgatgtgccctctgcgccgcggctgagacagcgggaaccggccccgggaggagccgcagcctgagcggccgactgaggaggcgaaggatgggcggggccacagggtcgacgac

SEQ ID NO: 16389 - RNA, 3323 nt, Homo sapiens
  source 1..3323: mol_type = other RNA
gtccacttctgcctgccctgccctaccctccccctttgggtttgtttgaggtttcattccacaaataagcagcagataaaatactttacaaggtacagcacagttgtattgaagaaaaaaaggacccaactcttactttaggagtattaggcctggacttcccctgccccatgcaataaagcaagttttatatacactccccatatttttttctaacattttcttatataaatttaaatattttacaaaaaaaggcttttttcctccaaacatataaatctgagtgaaacatagattccccacccgagaacttgtttcttcactaaaatataaatgttgtctgatattaagggtaaatgtcttttgaccactggagatcactgaagtctgaattgcaccgtggagaaggcacttgtgttttctgaggtctccagcaagtatctcagtgagcactcatagaattgctgtctgtcctccagaacccgtgccaaggcctccgagtgcccagttactgaggcagctggggaaaaacgttgagtaaacatgattctacaattacggagataaaaaataaaaacagcatggactggttctaccctagaatcaaactacaacaaaatccaaagtgttcattcatgtagattcaaaatgacttcattctgtcataaattataaaatacaaaggtggctgttttaatgacaaaactcaaaacagtactaaaaggggtttgtgtcaatggacaaaagtcagtccctctaggtagggccccaaggagcatcacccaggttgaagggtggttttcctactgctgggccagaagtgctgtcctattggccttcatcttctccagccgcttggccaggtggctgttggtcatctccatctcctcaatcttgtccagtgctgttcgtaactctcgttgtagcttccgtttttctgctttcaattcatcttcaactttctcagcattctcagcagcagttttatatctcagaacctgtccctcaagccggctaatactttgctccaaggtagttatatcctgttctgcttttgaaagcttaaatttgtattcgctaatttgtctattggcatctctctgcatttcgatgaactgcaagtctgagccattctgcagtcctgccaggtcacccactgtgccatcattcctggagcatttctgtcgttcctcctctaactgaagcttcagttttctaatctgtgacagtagttcttccttctctccagcaagttttcgtagccttacatctaatggcccttctcctgctgactccaagacctgagcagcttcctgagacacaacagtgatggctccagccactggttcatgactgacatcaccattgggagtgccatcggggattataactaagccatgtttctctcccgtcttcactgtctcctgcaggtcagccagctcctctctgagcatatctcgctcattcctaaggcaggcaatgtattctttctgtttctctagggccccaatttttttatctttccaaagaagtgtctcctggaggtcaaacacctcttttgtcatggtgtctattttctgctgcatgcgctgcttctcctcaataagctcatctctttgccgcaggccttctttaagttcttccatcttatgctgcagcacactacacatatgtttctgcctttctaactcctttgatttttcttcattttctctataaaattctgccatctgttcctcctgctcttcaataacatccttgagtgtgtctacttggtagatcaaattgttcttctcattgtctaactgtgcattggaaaccatggctttcttgtatttttcttccacttcagacaaagattcccgcaattcacttaatgaagtgtctggatctattaagctgctggtgtccccacttcctcgtctggatgagtttccacttagaggggttgttgctgaggcagaatttcgagatgaaggtcttgtataattttcagcatactgtttgtcagatttttcatccaactctttttgttgtcgttccagttctctcatgcgtatatctcttgcttctgcccgggcagcccgttttgctgccagccttgcctctgcctctctggcaatgttactcaaagcttcatcttctgcagaaaatcggtctttcacaggtgttcttttccttccagaagcaggagtccccatcttgtgttcttaatagtcttttaactttgaaagtgatttaactgtgttttcagcccttagtgatggtagctctcctttccactgacatttacatctagaccccttcatttatcttcccacatcttttccccagcgcggtggaagggtgagcgttagaaatcagacgggatgtctgagaacgccgcaggcagggggcgaccccagcccgggagcccgccgcgggccggccagtccccagggaagcccggccccctagccgaggtcggaggcggcgcggatcccacgggactgcggaggccgggaaaaaggttcccaactccccgctccctgctcccaccgggctggcgggaggagcggcccttacctgtgttagggcgcgcgctgcgactgcgtcgctgtccgggaagggccgaagagctgctcgcccgcccggcgcccgctggggctatgggcgaggggcgcagctggacgactcagtcctgggtccccggccaggcgggcggggatggacgcggcggctcccggcactggcagccggctagtcggtcaggccgatgtgccctctgcgccgcggctgagacagcgggaaccggccccgggaggagccgcagcctgagcggccgactgaggaggcgaaggatgggcggggccacagggtcgacgacccactcacccggaagcagttgtggccgcgactgcccgggagtggcgcttgccgcggtccgggcttgcaccccgctgggcaaagtacccggggctgtcacacggcgagctgagccctgggccggcgggtgaggttccccaagcggcgatgcccctggctccctgttccgccattgcgagccgttagggccaagctggagggagggcggcgaggcgcggctgccggtagggcggggccctgggctgctggcggggcggaggccggaggcggccttgggcgggtggcttctctgggtcccacggttcctgcccaggctcttcgaaccaggaccagtgcgggtaatgtgaattgacacttgttccggttcagggctgccccacccctggttgccccaaaccctgcggcctggtgggcttgggcaagtgggctggagtagcgctctgttaggaaacgagtat

SEQ ID NO: 16390 - RNA, 3287 nt, Homo sapiens
  source 1..3287: mol_type = other RNA
gtccacttctgcctgccctgccctaccctccccctttgggtttgtttgaggtttcattccacaaataagcagcagataaaatactttacaaggtacagcacagttgtattgaagaaaaaaaggacccaactcttactttaggagtattaggcctggacttcccctgccccatgcaataaagcaagttttatatacactccccatatttttttctaacattttcttatataaatttaaatattttacaaaaaaaggcttttttcctccaaacatataaatctgagtgaaacatagattccccacccgagaacttgtttcttcactaaaatataaatgttgtctgatattaagggtaaatgtcttttgaccactggagatcactgaagtctgaattgcaccgtggagaaggcacttgtgttttctgaggtctccagcaagtatctcagtgagcactcatagaattgctgtctgtcctccagaacccgtgccaaggcctccgagtgcccagttactgaggcagctggggaaaaacgttgagtaaacatgattctacaattacggagataaaaaataaaaacagcatggactggttctaccctagaatcaaactacaacaaaatccaaagtgttcattcatgtagattcaaaatgacttcattctgtcataaattataaaatacaaaggtggctgttttaatgacaaaactcaaaacagtactaaaaggggtttgtgtcaatggacaaaagtcagtccctctaggtagggccccaaggagcatcacccaggttgaagggtggttttcctactgctgggccagaagtgctgtcctattggccttcatcttctccagccgcttggccaggtggctgttggtcatctccatctcctcaatcttgtccagtgctgttcgtaactctcgttgtagcttccgtttttctgctttcaattcatcttcaactttctcagcattctcagcagcagttttatatctcagaacctgtccctcaagccggctaatactttgctccaaggtagttatatcctgttctgcttttgaaagcttaaatttgtattcgctaatttgtctattggcatctctctgcatttcgatgaactgcaagtctgagccattctgcagtcctgccaggtcacccactgtgccatcattcctggagcatttctgtcgttcctcctctaactgaagcttcagttttctaatctgtgacagtagttcttccttctctccagcaagttttcgtagccttacatctaatggcccttctcctgctgactccaagacctgagcagcttcctgagacacaacagtgatggctccagccactggttcatgactgacatcaccattgggagtgccatcggggattataactaagccatgtttctctcccgtcttcactgtctcctgcaggtcagccagctcctctctgagcatatctcgctcattcctaaggcaggcaatgtattctttctgtttctctagggccccaatttttttatctttccaaagaagtgtctcctggaggtcaaacacctcttttgtcatggtgtctattttctgctgcatgcgctgcttctcctcaataagctcatctctttgccgcaggccttctttaagttcttccatcttatgctgcagcacactacacatatgtttctgcctttctaactcctttgatttttcttcattttctctataaaattctgccatctgttcctcctgctcttcaataacatccttgagtgtgtctacttggtagatcaaattgttcttctcattgtctaactgtgcattggaaaccatggctttcttgtatttttcttccacttcagacaaagattcccgcaattcacttaatgaagtgtctggatctattaagctgctggtgtccccacttcctcgtctggatgagtttccacttagaggggttgttgctgaggcagaatttcgagatgaaggtcttgtataattttcagcatactgtttgtcagatttttcatccaagctggacaaatctgggatactgatatcatccacctcagagacaacacttcccctacgattggagcgactgaaataatcagcggcagataccacactctcccttcgtccacgactggcacgatcagaagacacaatgcttgcagtgtcatcgttggtaaaccctggactgcttcgggctgaacttattcttgatgaataataactgcattcagatggagttcgaggaccataagggttatataatccaccattgtacaatgatgccagactggcacttctcagcagaccagaatttgcagtaggagaggccctgtcactcttatatgttgccagagggtcactgtacagggaagaagactgccgagtgtagtaggcagaggtgggtttgctatgtctaagactgctatagtttctctggtcaaagtagaggccactcagtaggtctttatgagaatcagaagacctcttcttcattccatgagagtgactgtaagaatgatttaatgatgaaagtcttgatgatctatccttgaacatatcatacctgtgactgccaacacttcgaatggacaatgcatcctcaactcccagataaggacgatggtgactggaccggtgggaatacctggccctttccgaatcttccagccacttctgaatctgtccccacttccgatcaaaggaatgaagagagtactctttttgttgtcgttccagttctctcatgcgtatatctcttgcttctgcccgggcagcccgttttgctgccagccttgcctctgcctctctggcaatgttactcaaagcttcatcttctgcagaaaatcggtctttcacaggtgttcttttccttccagaagcaggagtccccatcttgtgttcttaatagtcttttaactttgaaagtgatttaactgtgttttcagcccttagtgatggtagctctcctttccactgacatttacatctagaccccttcatttatcttcccacatctgtgttagggcgcgcgctgcgactgcgtcgctgtccgggaagggccgaagagctgctcgcccgcccggcgcccgctggggctatgggcgaggggcgcagctggacgactcagtcctgggtccccggccaggcgggcggggatggacgcggcggctcccggcactggcagccggctagtcggtcaggccgatgtgccctctgcgccgcggctgagacagcgggaaccggccccgggaggagccgcagcctgagcggccgactgaggag

SEQ ID NO: 16391 - RNA, 3143 nt, Homo sapiens
  source 1..3143: mol_type = other RNA
gtccacttctgcctgccctgccctaccctccccctttgggtttgtttgaggtttcattccacaaataagcagcagataaaatactttacaaggtacagcacagttgtattgaagaaaaaaaggacccaactcttactttaggagtattaggcctggacttcccctgccccatgcaataaagcaagttttatatacactccccatatttttttctaacattttcttatataaatttaaatattttacaaaaaaaggcttttttcctccaaacatataaatctgagtgaaacatagattccccacccgagaacttgtttcttcactaaaatataaatgttgtctgatattaagggtaaatgtcttttgaccactggagatcactgaagtctgaattgcaccgtggagaaggcacttgtgttttctgaggtctccagcaagtatctcagtgagcactcatagaattgctgtctgtcctccagaacccgtgccaaggcctccgagtgcccagttactgaggcagctggggaaaaacgttgagtaaacatgattctacaattacggagataaaaaataaaaacagcatggactggttctaccctagaatcaaactacaacaaaatccaaagtgttcattcatgtagattcaaaatgacttcattctgtcataaattataaaatacaaaggtggctgttttaatgacaaaactcaaaacagtactaaaaggggtttgtgtcaatggacaaaagtcagtccctctaggtagggccccaaggagcatcacccaggttgaagggtggttttcctactgctgggccagaagtgctgtcctattggccttcatcttctccagccgcttggccaggtggctgttggtcatctccatctcctcaatcttgtccagtgctgttcgtaactctcgttgtagcttccgtttttctgctttcaattcatcttcaactttctcagcattctcagcagcagttttatatctcagaacctgtccctcaagccggctaatactttgctccaaggtagttatatcctgttctgcttttgaaagcttaaatttgtattcgctaatttgtctattggcatctctctgcatttcgatgaactgcaagtctgagccattctgcagtcctgccaggtcacccactgtgccatcattcctggagcatttctgtcgttcctcctctaactgaagcttcagttttctaatctgtgacagtagttcttccttctctccagcaagttttcgtagccttacatctaatggcccttctcctgctgactccaagacctgagcagcttcctgagacacaacagtgatggctccagccactggttcatgactgacatcaccattgggagtgccatcggggattataactaagccatgtttctctcccgtcttcactgtctcctgcaggtcagccagctcctctctgagcatatctcgctcattcctaaggcaggcaatgtattctttctgtttctctagggccccaatttttttatctttccaaagaagtgtctcctggaggtcaaacacctcttttgtcatggtgtctattttctgctgcatgcgctgcttctcctcaataagctcatctctttgccgcaggccttctttaagttcttccatcttatgctgcagcacactacacatatgtttctgcctttctaactcctttgatttttcttcattttctctataaaattctgccatctgttcctcctgctcttcaataacatccttgagtgtgtctacttggtagatcaaattgttcttctcattgtctaactgtgcattggaaaccatggctttcttgtatttttcttccacttcagacaaagattcctttagttctttaagcccctgcatgtatctcccttctacatcctgtatctggtccttaaggtcatagatatcccgcaattcacttaatgaagtgtctggatctattaagctgctggtgtccccacttcctcgtctggatgagtttccacttagaggggttgttgctgaggcagaatttcgagatgaaggtcttgtataattttcagcatactgtttgtcagatttttcatccaaagttcgaggaccataagggttatataatccaccattgtacaatgatgccagactggcacttctcagcagaccagaatttgcagtaggagaggccctgtcactcttatatgttgccagagggtcactgtacagggaagaagactgccgagtgtagtaggcagaggtgggtttgctatgtctaagactgctatagtttctctggtcaaagtagaggccactcagtaggtctttatgagaatcagaagacctcttcttcattccatgagagtgactgtaagaatgatttaatgatgaaagtcttgatgatctatccttgaacatatcatacctgtgactgccaacacttcgaatggacaatgcatcctcaactcccagataaggacgatggtgactggaccggtgggaatacctggccctttccgaatcttccagccacttctgaatctgtccccacttccgatcaaaggaatgaagagagtactctttttgttgtcgttccagttctctcatgcgtatatctcttgcttctgcccgggcagcccgttttgctgccagccttgcctctgcctctctggcaatgttactcaaagcttcatcttctgcagaaaatcggtctttcacaggtgttcttttccttccagaagcaggagtccccatcttgtgttcttaatagtcttttaactttgaaagtgatttaactgtgttttcagcccttagtgatggtagctctcctttccactgacatttacatctagaccccttcatttatcttcccacatctgtgttagggcgcgcgctgcgactgcgtcgctgtccgggaagggccgaagagctgctcgcccgcccggcgcccgctggggctatgggcgaggggcgcagctggacgactcagtcctgggtccccggccaggcgggcggggatggacgcggcggctcccggcactggcagccggctagtcggtcaggccgatgtgccctctgcgccgcggctgagacagcgggaaccggccccgggaggagccgcagcctgagcggccgactgaggag

SEQ ID NO: 16392 - RNA, 3269 nt, Homo sapiens
  source 1..3269: mol_type = other RNA
gtccacttctgcctgccctgccctaccctccccctttgggtttgtttgaggtttcattccacaaataagcagcagataaaatactttacaaggtacagcacagttgtattgaagaaaaaaaggacccaactcttactttaggagtattaggcctggacttcccctgccccatgcaataaagcaagttttatatacactccccatatttttttctaacattttcttatataaatttaaatattttacaaaaaaaggcttttttcctccaaacatataaatctgagtgaaacatagattccccacccgagaacttgtttcttcactaaaatataaatgttgtctgatattaagggtaaatgtcttttgaccactggagatcactgaagtctgaattgcaccgtggagaaggcacttgtgttttctgaggtctccagcaagtatctcagtgagcactcatagaattgctgtctgtcctccagaacccgtgccaaggcctccgagtgcccagttactgaggcagctggggaaaaacgttgagtaaacatgattctacaattacggagataaaaaataaaaacagcatggactggttctaccctagaatcaaactacaacaaaatccaaagtgttcattcatgtagattcaaaatgacttcattctgtcataaattataaaatacaaaggtggctgttttaatgacaaaactcaaaacagtactaaaaggggtttgtgtcaatggacaaaagtcagtccctctaggtagggccccaaggagcatcacccaggttgaagggtggttttcctactgctgggccagaagtgctgtcctattggccttcatcttctccagccgcttggccaggtggctgttggtcatctccatctcctcaatcttgtccagtgctgttcgtaactctcgttgtagcttccgtttttctgctttcaattcatcttcaactttctcagcattctcagcagcagttttatatctcagaacctgtccctcaagccggctaatactttgctccaaggtagttatatcctgttctgcttttgaaagcttaaatttgtattcgctaatttgtctattggcatctctctgcatttcgatgaactgcaagtctgagccattctgcagtcctgccaggtcacccactgtgccatcattcctggagcatttctgtcgttcctcctctaactgaagcttcagttttctaatctgtgacagtagttcttccttctctccagcaagttttcgtagccttacatctaatggcccttctcctgctgactccaagacctgagcagcttcctgagacacaacagtgatggctccagccactggttcatgactgacatcaccattgggagtgccatcggggattataactaagccatgtttctctcccgtcttcactgtctcctgcaggtcagccagctcctctctgagcatatctcgctcattcctaaggcaggcaatgtattctttctgtttctctagggccccaatttttttatctttccaaagaagtgtctcctggaggtcaaacacctcttttgtcatggtgtctattttctgctgcatgcgctgcttctcctcaataagctcatctctttgccgcaggccttctttaagttcttccatcttatgctgcagcacactacacatatgtttctgcctttctaactcctttgatttttcttcattttctctataaaattctgccatctgttcctcctgctcttcaataacatccttgagtgtgtctacttggtagatcaaattgttcttctcattgtctaactgtgcattggaaaccatggctttcttgtatttttcttccacttcagacaaagattcctttagttctttaagcccctgcatgtatctcccttctacatcctgtatctggtccttaaggtcatagatatcccgcaattcacttaatgaagtgtctggatctattaagctgctggtgtccccacttcctcgtctggatgagtttccacttagaggggttgttgctgaggcagaatttcgagatgaaggtcttgtataattttcagcatactgtttgtcagatttttcatccaacacactctcccttcgtccacgactggcacgatcagaagacacaatgcttgcagtgtcatcgttggtaaaccctggactgcttcgggctgaacttattcttgatgaataataactgcattcagatggagttcgaggaccataagggttatataatccaccattgtacaatgatgccagactggcacttctcagcagaccagaatttgcagtaggagaggccctgtcactcttatatgttgccagagggtcactgtacagggaagaagactgccgagtgtagtaggcagaggtgggtttgctatgtctaagactgctatagtttctctggtcaaagtagaggccactcagtaggtctttatgagaatcagaagacctcttcttcattccatgagagtgactgtaagaatgatttaatgatgaaagtcttgatgatctatccttgaacatatcatacctgtgactgccaacacttcgaatggacaatgcatcctcaactcccagataaggacgatggtgactggaccggtgggaatacctggccctttccgaatcttccagccacttctgaatctgtccccacttccgatcaaaggaatgaagagagtactctttttgttgtcgttccagttctctcatgcgtatatctcttgcttctgcccgggcagcccgttttgctgccagccttgcctctgcctctctggcaatgttactcaaagcttcatcttctgcagaaaatcggtctttcacaggtgttcttttccttccagaagcaggagtccccatcttgtgttcttaatagtcttttaactttgaaagtgatttaactgtgttttcagcccttagtgatggtagctctcctttccactgacatttacatctagaccccttcatttatcttcccacatctgtgttagggcgcgcgctgcgactgcgtcgctgtccgggaagggccgaagagctgctcgcccgcccggcgcccgctggggctatgggcgaggggcgcagctggacgactcagtcctgggtccccggccaggcgggcggggatggacgcggcggctcccggcactggcagccggctagtcggtcaggccgatgtgccctctgcgccgcggctgagacagcgggaaccggccccgggaggagccgcagcctgagcggccgactgaggag

SEQ ID NO: 16393 - RNA, 3902 nt, Homo sapiens
  source 1..3902: mol_type = other RNA
gtccacttctgcctgccctgccctaccctccccctttgggtttgtttgaggtttcattccacaaataagcagcagataaaatactttacaaggtacagcacagttgtattgaagaaaaaaaggacccaactcttactttaggagtattaggcctggacttcccctgccccatgcaataaagcaagttttatatacactccccatatttttttctaacattttcttatataaatttaaatattttacaaaaaaaggcttttttcctccaaacatataaatctgagtgaaacatagattccccacccgagaacttgtttcttcactaaaatataaatgttgtctgatattaagggtaaatgtcttttgaccactggagatcactgaagtctgaattgcaccgtggagaaggcacttgtgttttctgaggtctccagcaagtatctcagtgagcactcatagaattgctgtctgtcctccagaacccgtgccaaggcctccgagtgcccagttactgaggcagctggggaaaaacgttgagtaaacatgattctacaattacggagataaaaaataaaaacagcatggactggttctaccctagaatcaaactacaacaaaatccaaagtgttcattcatgtagattcaaaatgacttcattctgtcataaattataaaatacaaaggtggctgttttaatgacaaaactcaaaacagtactaaaaggggtttgtgtcaatggacaaaagtcagtccctctaggtagggccccaaggagcatcacccaggttgaagggtggttttcctactgctgggccagaagtgctgtcctattggccttcatcttctccagccgcttggccaggtggctgttggtcatctccatctcctcaatcttgtccagtgctgttcgtaactctcgttgtagcttccgtttttctgctttcaattcatcttcaactttctcagcattctcagcagcagttttatatctcagaacctgtccctcaagccggctaatactttgctccaaggtagttatatcctgttctgcttttgaaagcttaaatttgtattcgctaatttgtctattggcatctctctgcatttcgatgaactgcaagtctgagccattctgcagtcctgccaggtcacccactgtgccatcattcctggagcatttctgtcgttcctcctctaactgaagcttcagttttctaatctgtgacagtagttcttccttctctccagcaagttttcgtagccttacatctaatggcccttctcctgctgactccaagacctgagcagcttcctgagacacaacagtgatggctccagccactggttcatgactgacatcaccattgggagtgccatcggggattataactaagccatgtttctctcccgtcttcactgtctcctgcaggtcagccagctcctctctgagcatatctcgctcattcctaaggcaggcaatgtattctttctgtttctctagggccccaatttttttatctttccaaagaagtgtctcctggaggtcaaacacctcttttgtcatggtgtctattttctgctgcatgcgctgcttctcctcaataagctcatctctttgccgcaggccttctttaagttcttccatcttatgctgcagcacactacacatatgtttctgcctttctaactcctttgatttttcttcattttctctataaaattctgccatctgttcctcctgctcttcaataacatccttgagtgtgtctacttggtagatcaaattgttcttctcattgtctaactgtgcattggaaaccatggctttcttgtatttttcttccacttcagacaaagattcctttagttctttaagcccctgcatgtatctcccttctacatcctgtatctggtccttaaggtcatagatatcccgcaattcacttaatgaagtgtctggatctattaagctgctggtgtccccacttcctcgtctggatgagtttccacttagaggggttgttgctgaggcagaatttcgagatgaaggtcttgtataattttcagcatactgtttgtcagatttttcatccaacacactctcccttcgtccacgactggcacgatcagaagacacaatgcttgcagtgtcatcgttggtaaaccctggactgcttcgggctgaacttattcttgatgaataataactgcattcagatggagttcgaggaccataagggttatataatccaccattgtacaatgatgccctgtcactcttatatgttgccagagggtcactgtacagggaagaagaccgagtgtagtaggcagaggtgggtttgctatgtctaagactgctatagtttctctggtcaaagtagaggccactcagtaggtctttatgagaatcagaagacctcttcttcattccatgagagtgactgtaagaatgatttaatgatgaaagtcttgatgatctatccttgaacatatcatacctgtgactgccaacacttcgaatggacaatgcatcctcaactcccagataaggacgatggtgactggaccggtgggaatacctggccctttccgaatcttcctctttttgttgtcgttccagttctctcatgcgtatatctcttgcttctgcccgggcagcccgttttgctgccagccttgcctctgcctctctggcaatgttactcaaagcttcatcttctgcagaaaatcggtctttcacaggtgttcttttccttccagaagcaggagtccccatcttgtgttcttaatagtcttttaactttgaaagtgatttaactgtgttttcagcccttagtgatggtagctctcctttccactgacatttacatctagaccccttcatttatcttcccacatcttttccccagcgcggtggaagggtgagcgttagaaatcagacgggatgtctgagaacgccgcaggcagggggcgaccccagcccgggagcccgccgcgggccggccagtccccagggaagcccggccccctagccgaggtcggaggcggcgcggatcccacgggactgcggaggccgggaaaaaggttcccaactccccgctccctgctcccaccgggctggcgggaggagcggcccttacctgtgttagggcgcgcgctgcgactgcgtcgctgtccgggaagggccgaagagctgctcgcccgcccggcgcccgctggggctatgggcgaggggcgcagctggacgactcagtcctgggtccccggccaggcgggcggggatggacgcggcggctcccggcactggcagccggctagtcggtcaggccgatgtgccctctgcgccgcggctgagacagcgggaaccggccccgggaggagccgcagcctgagcggccgactgaggaggcgaaggatgggcggggccacagggtcgacgacccactcacccggaagcagttgtggccgcgactgcccgggagtggcgcttgccgcggtccgggcttgcaccccgctgggcaaagtacccggggctgtcacacggcgagctgagccctgggccggcgggtgaggttccccaagcggcgatgcccctggctccctgttccgccattgcgagccgttagggccaagctggagggagggcggcgaggcgcggctgccggtagggcggggccctgggctgctggcggggcggaggccggaggcggccttgggcgggtggcttctctgggtcccacggttcctgcccaggctcttcgaaccaggaccagtgcgggtaatgtgaattgacacttgttccggttcagggctgccccacccctggttgccccaaaccctgcggcctggtgggcttgggcaagtgggctggagtagcgctctgttaggaaacgagtat

SEQ ID NO: 16394 - RNA, 3200 nt, Homo sapiens
  source 1..3200: mol_type = other RNA
gtccacttctgcctgccctgccctaccctccccctttgggtttgtttgaggtttcattccacaaataagcagcagataaaatactttacaaggtacagcacagttgtattgaagaaaaaaaggacccaactcttactttaggagtattaggcctggacttcccctgccccatgcaataaagcaagttttatatacactccccatatttttttctaacattttcttatataaatttaaatattttacaaaaaaaggcttttttcctccaaacatataaatctgagtgaaacatagattccccacccgagaacttgtttcttcactaaaatataaatgttgtctgatattaagggtaaatgtcttttgaccactggagatcactgaagtctgaattgcaccgtggagaaggcacttgtgttttctgaggtctccagcaagtatctcagtgagcactcatagaattgctgtctgtcctccagaacccgtgccaaggcctccgagtgcccagttactgaggcagctggggaaaaacgttgagtaaacatgattctacaattacggagataaaaaataaaaacagcatggactggttctaccctagaatcaaactacaacaaaatccaaagtgttcattcatgtagattcaaaatgacttcattctgtcataaattataaaatacaaaggtggctgttttaatgacaaaactcaaaacagtactaaaaggggtttgtgtcaatggacaaaagtcagtccctctaggtagggccccaaggagcatcacccaggttgaagggtggttttcctactgctgggccagaagtgctgtcctattggccttcatcttctccagccgcttggccaggtggctgttggtcatctccatctcctcaatcttgtccagtgctgttcgtaactctcgttgtagcttccgtttttctgctttcaattcatcttcaactttctcagcattctcagcagcagttttatatctcagaacctgtccctcaagccggctaatactttgctccaaggtagttatatcctgttctgcttttgaaagcttaaatttgtattcgctaatttgtctattggcatctctctgcatttcgatgaactgcaagtctgagccattctgcagtcctgccaggtcacccactgtgccatcattcctggagcatttctgtcgttcctcctctaactgaagcttcagttttctaatctgtgacagtagttcttccttctctccagcaagttttcgtagccttacatctaatggcccttctcctgctgactccaagacctgagcagcttcctgagacacaacagtgatggctccagccactggttcatgactgacatcaccattgggagtgccatcggggattataactaagccatgtttctctcccgtcttcactgtctcctgcaggtcagccagctcctctctgagcatatctcgctcattcctaaggcaggcaatgtattctttctgtttctctagggccccaatttttttatctttccaaagaagtgtctcctggaggtcaaacacctcttttgtcatggtgtctattttctgctgcatgcgctgcttctcctcaataagctcatctctttgccgcaggccttctttaagttcttccatcttatgctgcagcacactacacatatgtttctgcctttctaactcctttgatttttcttcattttctctataaaattctgccatctgttcctcctgctcttcaataacatccttgagtgtgtctacttggtagatcaaattgttcttctcattgtctaactgtgcattggaaaccatggctttcttgtatttttcttccacttcagacaaagattcctttagttctttaagcccctgcatgtatctcccttctacatcctgtatctggtccttaaggtcatagatatcccgcaattcacttaatgaagtgtctggatctattaagctgctggtgtccccacttcctcgtctggatgagtttccacttagaggggttgttgctgaggcagaatttcgagatgaaggtcttgtataattttcagcatactgtttgtcagatttttcatccaaccctggactgcttcgggctgaacttattcttgatgaataataactgcattcagatggagttcgaggaccataagggttatataatccaccattgtacaatgatgccagactggcacttctcagcagaccagaatttgcagtaggagaggccctgtcactcttatatgttgccagagggtcactgtacagggaagaagactgccgagtgtagtaggcagaggtgggtttgctatgtctaagactgctatagtttctctggtcaaagtagaggccactcagtaggtctttatgagaatcagaagacctcttcttcattccatgagagtgactgtaagaatgatttaatgatgaaagtcttgatgatctatccttgaacatatcatacctgtgactgccaacacttcgaatggacaatgcatcctcaactcccagataaggacgatggtgactggaccggtgggaatacctggccctttccgaatcttccagccacttctgaatctgtccccacttccgatcaaaggaatgaagagagtactctttttgttgtcgttccagttctctcatgcgtatatctcttgcttctgcccgggcagcccgttttgctgccagccttgcctctgcctctctggcaatgttactcaaagcttcatcttctgcagaaaatcggtctttcacaggtgttcttttccttccagaagcaggagtccccatcttgtgttcttaatagtcttttaactttgaaagtgatttaactgtgttttcagcccttagtgatggtagctctcctttccactgacatttacatctagaccccttcatttatcttcccacatctgtgttagggcgcgcgctgcgactgcgtcgctgtccgggaagggccgaagagctgctcgcccgcccggcgcccgctggggctatgggcgaggggcgcagctggacgactcagtcctgggtccccggccaggcgggcggggatggacgcggcggctcccggcactggcagccggctagtcggtcaggccgatgtgccctctgcgccgcggctgagacagcgggaaccggccccgggaggagccgcagcctgagcggccgactgaggag

SEQ ID NO: 16395 - RNA, 2816 nt, Homo sapiens
  source 1..2816: mol_type = other RNA
gtccacttctgcctgccctgccctaccctccccctttgggtttgtttgaggtttcattccacaaataagcagcagataaaatactttacaaggtacagcacagttgtattgaagaaaaaaaggacccaactcttactttaggagtattaggcctggacttcccctgccccatgcaataaagcaagttttatatacactccccatatttttttctaacattttcttatataaatttaaatattttacaaaaaaaggcttttttcctccaaacatataaatctgagtgaaacatagattccccacccgagaacttgtttcttcactaaaatataaatgttgtctgatattaagggtaaatgtcttttgaccactggagatcactgaagtctgaattgcaccgtggagaaggcacttgtgttttctgaggtctccagcaagtatctcagtgagcactcatagaattgctgtctgtcctccagaacccgtgccaaggcctccgagtgcccagttactgaggcagctggggaaaaacgttgagtaaacatgattctacaattacggagataaaaaataaaaacagcatggactggttctaccctagaatcaaactacaacaaaatccaaagtgttcattcatgtagattcaaaatgacttcattctgtcataaattataaaatacaaaggtggctgttttaatgacaaaactcaaaacagtactaaaaggggtttgtgtcaatggacaaaagtcagtccctctaggtagggccccaaggagcatcacccaggttgaagggtggttttcctactgctgggccagaagtgctgtcctattggccttcatcttctccagccgcttggccaggtggctgttggtcatctccatctcctcaatcttgtccagtgctgttcgtaactctcgttgtagcttccgtttttctgctttcaattcatcttcaactttctcagcattctcagcagcagttttatatctcagaacctgtccctcaagccggctaatactttgctccaaggtagttatatcctgttctgcttttgaaagcttaaatttgtattcgctaatttgtctattggcatctctctgcatttcgatgaactgcaagtctgagccattctgcagtcctgccaggtcacccactgtgccatcattcctggagcatttctgtcgttcctcctctaactgaagcttcagttttctaatctgtgacagtagttcttccttctctccagcaagttttcgtagccttacatctaatggcccttctcctgctgactccaagacctgagcagcttcctgagacacaacagtgatggctccagccactggttcatgactgacatcaccattgggagtgccatcggggattataactaagccatgtttctctcccgtcttcactgtctcctgcaggtcagccagctcctctctgagcatatctcgctcattcctaaggcaggcaatgtattctttctgtttctctagggccccaatttttttatctttccaaagaagtgtctcctggaggtcaaacacctcttttgtcatggtgtctattttctgctgcatgcgctgcttctcctcaataagctcatctctttgccgcaggccttctttaagttcttccatcttatgctgcagcacactacacatatgtttctgcctttctaactcctttgatttttcttcattttctctataaaattctgccatctgttcctcctgctcttcaataacatccttgagtgtgtctacttggtagatcaaattgttcttctcattgtctaactgtgcattggaaaccatggctttcttgtatttttcttccacttcagacaaagattcctttagttctttaagcccctgcatgtatctcccttctacatcctgtatctggtccttaaggtcatagatatcccgcaattcacttaatgaagtgtctggatctattaagctgctggtgtccccacttcctcgtctggatgagtttccacttagaggggttgttgctgaggcagaatttcgagatgaaggtcttgtataattttcagcatactgtttgtcagatttttcatccaacctgtgactgccaacacttcgaatggacaatgcatcctcaactcccagataaggacgatggtgactggaccggtgggaatacctggccctttccgaatcttccagccacttctgaatctgtccccacttccgatcaaaggaatgaagagagtactctttttgttgtcgttccagttctctcatgcgtatatctcttgcttctgcccgggcagcccgttttgctgccagccttgcctctgcctctctggcaatgttactcaaagcttcatcttctgcagaaaatcggtctttcacaggtgttcttttccttccagaagcaggagtccccatcttgtgttcttaatagtcttttaactttgaaagtgatttaactgtgttttcagcccttagtgatggtagctctcctttccactgacatttacatctagaccccttcatttatcttcccacatctgtgttagggcgcgcgctgcgactgcgtcgctgtccgggaagggccgaagagctgctcgcccgcccggcgcccgctggggctatgggcgaggggcgcagctggacgactcagtcctgggtccccggccaggcgggcggggatggacgcggcggctcccggcactggcagccggctagtcggtcaggccgatgtgccctctgcgccgcggctgagacagcgggaaccggccccgggaggagccgcagcctgagcggccgactgaggag

SEQ ID NO: 16396 - RNA, 2765 nt, Homo sapiens
  source 1..2765: mol_type = other RNA
gtccacttctgcctgccctgccctaccctccccctttgggtttgtttgaggtttcattccacaaataagcagcagataaaatactttacaaggtacagcacagttgtattgaagaaaaaaaggacccaactcttactttaggagtattaggcctggacttcccctgccccatgcaataaagcaagttttatatacactccccatatttttttctaacattttcttatataaatttaaatattttacaaaaaaaggcttttttcctccaaacatataaatctgagtgaaacatagattccccacccgagaacttgtttcttcactaaaatataaatgttgtctgatattaagggtaaatgtcttttgaccactggagatcactgaagtctgaattgcaccgtggagaaggcacttgtgttttctgaggtctccagcaagtatctcagtgagcactcatagaattgctgtctgtcctccagaacccgtgccaaggcctccgagtgcccagttactgaggcagctggggaaaaacgttgagtaaacatgattctacaattacggagataaaaaataaaaacagcatggactggttctaccctagaatcaaactacaacaaaatccaaagtgttcattcatgtagattcaaaatgacttcattctgtcataaattataaaatacaaaggtggctgttttaatgacaaaactcaaaacagtactaaaaggggtttgtgtcaatggacaaaagtcagtccctctaggtagggccccaaggagcatcacccaggttgaagggtggttttcctactgctgggccagaagtgctgtcctattggccttcatcttctccagccgcttggccaggtggctgttggtcatctccatctcctcaatcttgtccagtgctgttcgtaactctcgttgtagcttccgtttttctgctttcaattcatcttcaactttctcagcattctcagcagcagttttatatctcagaacctgtccctcaagccggctaatactttgctccaaggtagttatatcctgttctgcttttgaaagcttaaatttgtattcgctaatttgtctattggcatctctctgcatttcgatgaactgcaagtctgagccattctgcagtcctgccaggtcacccactgtgccatcattcctggagcatttctgtcgttcctcctctaactgaagcttcagttttctaatctgtgacagtagttcttccttctctccagcaagttttcgtagccttacatctaatggcccttctcctgctgactccaagacctgagcagcttcctgagacacaacagtgatggctccagccactggttcatgactgacatcaccattgggagtgccatcggggattataactaagccatgtttctctcccgtcttcactgtctcctgcaggtcagccagctcctctctgagcatatctcgctcattcctaaggcaggcaatgtattctttctgtttctctagggccccaatttttttatctttccaaagaagtgtctcctggaggtcaaacacctcttttgtcatggtgtctattttctgctgcatgcgctgcttctcctcaataagctcatctctttgccgcaggccttctttaagttcttccatcttatgctgcagcacactacacatatgtttctgcctttctaactcctttgatttttcttcattttctctataaaattctgccatctgttcctcctgctcttcaataacatccttgagtgtgtctacttggtagatcaaattgttcttctcattgtctaactgtgcattggaaaccatggctttcttgtatttttcttccacttcagacaaagattcctttagttctttaagcccctgcatgtatctcccttctacatcctgtatctggtccttaaggtcatagatatcccgcaattcacttaatgaagtgtctggatctattaagctgctggtgtccccacttcctcgtctggatgagtttccacttagaggggttgttgctgaggcagaatttcgagatgaaggtcttgtataattttcagcatactgtttgtcagatttttcatccaacctgtgactgccaacacttcgaatggacaatgcatcctcaactcccagataaggacgatggtgactggaccggtgggaatacctggccctttccgaatcttcctctttttgttgtcgttccagttctctcatgcgtatatctcttgcttctgcccgggcagcccgttttgctgccagccttgcctctgcctctctggcaatgttactcaaagcttcatcttctgcagaaaatcggtctttcacaggtgttcttttccttccagaagcaggagtccccatcttgtgttcttaatagtcttttaactttgaaagtgatttaactgtgttttcagcccttagtgatggtagctctcctttccactgacatttacatctagaccccttcatttatcttcccacatctgtgttagggcgcgcgctgcgactgcgtcgctgtccgggaagggccgaagagctgctcgcccgcccggcgcccgctggggctatgggcgaggggcgcagctggacgactcagtcctgggtccccggccaggcgggcggggatggacgcggcggctcccggcactggcagccggctagtcggtcaggccgatgtgccctctgcgccgcggctgagacagcgggaaccggccccgggaggagccgcagcctgagcggccgactgaggag

SEQ ID NO: 16397 - RNA, 2751 nt, Homo sapiens
  source 1..2751: mol_type = other RNA
gtccacttctgcctgccctgccctaccctccccctttgggtttgtttgaggtttcattccacaaataagcagcagataaaatactttacaaggtacagcacagttgtattgaagaaaaaaaggacccaactcttactttaggagtattaggcctggacttcccctgccccatgcaataaagcaagttttatatacactccccatatttttttctaacattttcttatataaatttaaatattttacaaaaaaaggcttttttcctccaaacatataaatctgagtgaaacatagattccccacccgagaacttgtttcttcactaaaatataaatgttgtctgatattaagggtaaatgtcttttgaccactggagatcactgaagtctgaattgcaccgtggagaaggcacttgtgttttctgaggtctccagcaagtatctcagtgagcactcatagaattgctgtctgtcctccagaacccgtgccaaggcctccgagtgcccagttactgaggcagctggggaaaaacgttgagtaaacatgattctacaattacggagataaaaaataaaaacagcatggactggttctaccctagaatcaaactacaacaaaatccaaagtgttcattcatgtagattcaaaatgacttcattctgtcataaattataaaatacaaaggtggctgttttaatgacaaaactcaaaacagtactaaaaggggtttgtgtcaatggacaaaagtcagtccctctaggtagggccccaaggagcatcacccaggttgaagggtggttttcctactgctgggccagaagtgctgtcctattggccttcatcttctccagccgcttggccaggtggctgttggtcatctccatctcctcaatcttgtccagtgctgttcgtaactctcgttgtagcttccgtttttctgctttcaattcatcttcaactttctcagcattctcagcagcagttttatatctcagaacctgtccctcaagccggctaatactttgctccaaggtagttatatcctgttctgcttttgaaagcttaaatttgtattcgctaatttgtctattggcatctctctgcatttcgatgaactgcaagtctgagccattctgcagtcctgccaggtcacccactgtgccatcattcctggagcatttctgtcgttcctcctctaactgaagcttcagttttctaatctgtgacagtagttcttccttctctccagcaagttttcgtagccttacatctaatggcccttctcctgctgactccaagacctgagcagcttcctgagacacaacagtgatggctccagccactggttcatgactgacatcaccattgggagtgccatcggggattataactaagccatgtttctctcccgtcttcactgtctcctgcaggtcagccagctcctctctgagcatatctcgctcattcctaaggcaggcaatgtattctttctgtttctctagggccccaatttttttatctttccaaagaagtgtctcctggaggtcaaacacctcttttgtcatggtgtctattttctgctgcatgcgctgcttctcctcaataagctcatctctttgccgcaggccttctttaagttcttccatcttatgctgcagcacactacacatatgtttctgcctttctaactcctttgatttttcttcattttctctataaaattctgccatctgttcctcctgctcttcaataacatccttgagtgtgtctacttggtagatcaaattgttcttctcattgtctaactgtgcattggaaaccatggctttcttgtatttttcttccacttcagacaaagattcctttagttctttaagcccctgcatgtatctcccttctacatcctgtatctggtccttaaggtcatagatatcccgcaattcacttaatgaagtgtctggatctattaagctgctggtgtccccacttcctcgtctggatgagtttccacttagaggggttgttgctgaggcagaatttcgagatgaaggtcttgtataattttcagcatactgtttgtcagatttttcatccaacctgtgactgccaacacttcgaatggacaatgcatcctcaactccctctttttgttgtcgttccagttctctcatgcgtatatctcttgcttctgcccgggcagcccgttttgctgccagccttgcctctgcctctctggcaatgttactcaaagcttcatcttctgcagaaaatcggtctttcacaggtgttcttttccttccagaagcaggagtccccatcttgtgttcttaatagtcttttaactttgaaagtgatttaactgtgttttcagccagaaaagaaggaaagtatcttcaggatcttgcagaatataaaccttagtgatggtagctctcctttccactgacatttacatctagaccccttcatttatcttcccacatctgtgttagggcgcgcgctgcgactgcgtcgctgtccgggaagggccgaagagctgctcgcccgcccggcgcccgctggggctatgggcgaggggcgcagctggacgactcagtcctgggtccccggccaggcgggcggggatggacgcggcggctcccggcactggcagccggctagtcggtcaggccgatgtgccctctgcgccgcggctgagacagcgggaaccggccccgggaggagccgcagcctgagcggccgactgaggag

SEQ ID NO: 16398 - RNA, 2708 nt, Homo sapiens
  source 1..2708: mol_type = other RNA
gtccacttctgcctgccctgccctaccctccccctttgggtttgtttgaggtttcattccacaaataagcagcagataaaatactttacaaggtacagcacagttgtattgaagaaaaaaaggacccaactcttactttaggagtattaggcctggacttcccctgccccatgcaataaagcaagttttatatacactccccatatttttttctaacattttcttatataaatttaaatattttacaaaaaaaggcttttttcctccaaacatataaatctgagtgaaacatagattccccacccgagaacttgtttcttcactaaaatataaatgttgtctgatattaagggtaaatgtcttttgaccactggagatcactgaagtctgaattgcaccgtggagaaggcacttgtgttttctgaggtctccagcaagtatctcagtgagcactcatagaattgctgtctgtcctccagaacccgtgccaaggcctccgagtgcccagttactgaggcagctggggaaaaacgttgagtaaacatgattctacaattacggagataaaaaataaaaacagcatggactggttctaccctagaatcaaactacaacaaaatccaaagtgttcattcatgtagattcaaaatgacttcattctgtcataaattataaaatacaaaggtggctgttttaatgacaaaactcaaaacagtactaaaaggggtttgtgtcaatggacaaaagtcagtccctctaggtagggccccaaggagcatcacccaggttgaagggtggttttcctactgctgggccagaagtgctgtcctattggccttcatcttctccagccgcttggccaggtggctgttggtcatctccatctcctcaatcttgtccagtgctgttcgtaactctcgttgtagcttccgtttttctgctttcaattcatcttcaactttctcagcattctcagcagcagttttatatctcagaacctgtccctcaagccggctaatactttgctccaaggtagttatatcctgttctgcttttgaaagcttaaatttgtattcgctaatttgtctattggcatctctctgcatttcgatgaactgcaagtctgagccattctgcagtcctgccaggtcacccactgtgccatcattcctggagcatttctgtcgttcctcctctaactgaagcttcagttttctaatctgtgacagtagttcttccttctctccagcaagttttcgtagccttacatctaatggcccttctcctgctgactccaagacctgagcagcttcctgagacacaacagtgatggctccagccactggttcatgactgacatcaccattgggagtgccatcggggattataactaagccatgtttctctcccgtcttcactgtctcctgcaggtcagccagctcctctctgagcatatctcgctcattcctaaggcaggcaatgtattctttctgtttctctagggccccaatttttttatctttccaaagaagtgtctcctggaggtcaaacacctcttttgtcatggtgtctattttctgctgcatgcgctgcttctcctcaataagctcatctctttgccgcaggccttctttaagttcttccatcttatgctgcagcacactacacatatgtttctgcctttctaactcctttgatttttcttcattttctctataaaattctgccatctgttcctcctgctcttcaataacatccttgagtgtgtctacttggtagatcaaattgttcttctcattgtctaactgtgcattggaaaccatggctttcttgtatttttcttccacttcagacaaagattcctttagttctttaagcccctgcatgtatctcccttctacatcctgtatctggtccttaaggtcatagatatcccgcaattcacttaatgaagtgtctggatctattaagctgctggtgtccccacttcctcgtctggatgagtttccacttagaggggttgttgctgaggcagaatttcgagatgaaggtcttgtataattttcagcatactgtttgtcagatttttcatccaacctgtgactgccaacacttcgaatggacaatgcatcctcaactccctctttttgttgtcgttccagttctctcatgcgtatatctcttgcttctgcccgggcagcccgttttgctgccagccttgcctctgcctctctggcaatgttactcaaagcttcatcttctgcagaaaatcggtctttcacaggtgttcttttccttccagaagcaggagtccccatcttgtgttcttaatagtcttttaactttgaaagtgatttaactgtgttttcagcccttagtgatggtagctctcctttccactgacatttacatctagaccccttcatttatcttcccacatctgtgttagggcgcgcgctgcgactgcgtcgctgtccgggaagggccgaagagctgctcgcccgcccggcgcccgctggggctatgggcgaggggcgcagctggacgactcagtcctgggtccccggccaggcgggcggggatggacgcggcggctcccggcactggcagccggctagtcggtcaggccgatgtgccctctgcgccgcggctgagacagcgggaaccggccccgggaggagccgcagcctgagcggccgactgaggag

SEQ ID NO: 16399 - RNA, 2706 nt, Homo sapiens
  source 1..2706: mol_type = other RNA
gtccacttctgcctgccctgccctaccctccccctttgggtttgtttgaggtttcattccacaaataagcagcagataaaatactttacaaggtacagcacagttgtattgaagaaaaaaaggacccaactcttactttaggagtattaggcctggacttcccctgccccatgcaataaagcaagttttatatacactccccatatttttttctaacattttcttatataaatttaaatattttacaaaaaaaggcttttttcctccaaacatataaatctgagtgaaacatagattccccacccgagaacttgtttcttcactaaaatataaatgttgtctgatattaagggtaaatgtcttttgaccactggagatcactgaagtctgaattgcaccgtggagaaggcacttgtgttttctgaggtctccagcaagtatctcagtgagcactcatagaattgctgtctgtcctccagaacccgtgccaaggcctccgagtgcccagttactgaggcagctggggaaaaacgttgagtaaacatgattctacaattacggagataaaaaataaaaacagcatggactggttctaccctagaatcaaactacaacaaaatccaaagtgttcattcatgtagattcaaaatgacttcattctgtcataaattataaaatacaaaggtggctgttttaatgacaaaactcaaaacagtactaaaaggggtttgtgtcaatggacaaaagtcagtccctctaggtagggccccaaggagcatcacccaggttgaagggtggttttcctactgctgggccagaagtgctgtcctattggccttcatcttctccagccgcttggccaggtggctgttggtcatctccatctcctcaatcttgtccagtgctgttcgtaactctcgttgtagcttccgtttttctgctttcaattcatcttcaactttctcagcattctcagcagcagttttatatctcagaacctgtccctcaagccggctaatactttgctccaaggtagttatatcctgttctgcttttgaaagcttaaatttgtattcgctaatttgtctattggcatctctctgcatttcgatgaactgcaagtctgagccattctgcagtcctgccaggtcacccactgtgccatcattcctggagcatttctgtcgttcctcctctaactgaagcttcagttttctaatctgtgacagtagttcttccttctctccagcaagttttcgtagccttacatctaatggcccttctcctgctgactccaagacctgagcagcttcctgagacacaacagtgatggctccagccactggttcatgactgacatcaccattgggagtgccatcggggattataactaagccatgtttctctcccgtcttcactgtctcctgcaggtcagccagctcctctctgagcatatctcgctcattcctaaggcaggcaatgtattctttctgtttctctagggccccaatttttttatctttccaaagaagtgtctcctggaggtcaaacacctcttttgtcatggtgtctattttctgctgcatgcgctgcttctcctcaataagctcatctctttgccgcaggccttctttaagttcttccatcttatgctgcagcacactacacatatgtttctgcctttctaactcctttgatttttcttcattttctctataaaattctgccatctgttcctcctgctcttcaataacatccttgagtgtgtctacttggtagatcaaattgttcttctcattgtctaactgtgcattggaaaccatggctttcttgtatttttcttccacttcagacaaagattcctttagttctttaagcccctgcatgtatctcccttctacatcctgtatctggtccttaaggtcatagatatcccgcaattcacttaatgaagtgtctggatctattaagctgctggtgtccccacttcctcgtctggatgagtttccacttagaggggttgttgctgaggcagaatttcgagatgaaggtcttgtataattttcagcatactgtttgtcagatttttcatccaactctttttgttgtcgttccagttctctcatgcgtatatctcttgcttctgcccgggcagcccgttttgctgccagccttgcctctgcctctctggcaatgttactcaaagcttcatcttctgcagaaaatcggtctttcacaggtgttcttttccttccagaagcaggagtccccatcttgtgttcttaatagtcttttaactttgaaagtgatttaactgtgttttcagccagaaaagaaggaaagtatcttcaggatcttgcagaatataaaccttagtgatggtagctctcctttccactgacatttacatctagaccccttcatttatcttcccacatctgtgttagggcgcgcgctgcgactgcgtcgctgtccgggaagggccgaagagctgctcgcccgcccggcgcccgctggggctatgggcgaggggcgcagctggacgactcagtcctgggtccccggccaggcgggcggggatggacgcggcggctcccggcactggcagccggctagtcggtcaggccgatgtgccctctgcgccgcggctgagacagcgggaaccggccccgggaggagccgcagcctgagcggccgactgaggag

SEQ ID NO: 16400 - RNA, 2696 nt, Homo sapiens
  source 1..2696: mol_type = other RNA
gtccacttctgcctgccctgccctaccctccccctttgggtttgtttgaggtttcattccacaaataagcagcagataaaatactttacaaggtacagcacagttgtattgaagaaaaaaaggacccaactcttactttaggagtattaggcctggacttcccctgccccatgcaataaagcaagttttatatacactccccatatttttttctaacattttcttatataaatttaaatattttacaaaaaaaggcttttttcctccaaacatataaatctgagtgaaacatagattccccacccgagaacttgtttcttcactaaaatataaatgttgtctgatattaagggtaaatgtcttttgaccactggagatcactgaagtctgaattgcaccgtggagaaggcacttgtgttttctgaggtctccagcaagtatctcagtgagcactcatagaattgctgtctgtcctccagaacccgtgccaaggcctccgagtgcccagttactgaggcagctggggaaaaacgttgagtaaacatgattctacaattacggagataaaaaataaaaacagcatggactggttctaccctagaatcaaactacaacaaaatccaaagtgttcattcatgtagattcaaaatgacttcattctgtcataaattataaaatacaaaggtggctgttttaatgacaaaactcaaaacagtactaaaaggggtttgtgtcaatggacaaaagtcagtccctctaggtagggccccaaggagcatcacccaggttgaagggtggttttcctactgctgggccagaagtgctgtcctattggccttcatcttctccagccgcttggccaggtggctgttggtcatctccatctcctcaatcttgtccagtgctgttcgtaactctcgttgtagcttccgtttttctgctttcaattcatcttcaactttctcagcattctcagcagcagttttatatctcagaacctgtccctcaagccggctaatactttgctccaaggtagttatatcctgttctgcttttgaaagcttaaatttgtattcgctaatttgtctattggcatctctctgcatttcgatgaactgcaagtctgagccattctgcagtcctgccaggtcacccactgtgccatcattcctggagcatttctgtcgttcctcctctaactgaagcttcagttttctaatctgtgacagtagttcttccttctctccagcaagttttcgtagccttacatctaatggcccttctcctgctgactccaagacctgagcagcttcctgagacacaacagtgatggctccagccactggttcatgactgacatcaccattgggagtgccatcggggattataactaagccatgtttctctcccgtcttcactgtctcctgcaggtcagccagctcctctctgagcatatctcgctcattcctaaggcaggcaatgtattctttctgtttctctagggccccaatttttttatctttccaaagaagtgtctcctggaggtcaaacacctcttttgtcatggtgtctattttctgctgcatgcgctgcttctcctcaataagctcatctctttgccgcaggccttctttaagttcttccatcttatgctgcagcacactacacatatgtttctgcctttctaactcctttgatttttcttcattttctctataaaattctgccatctgttcctcctgctcttcaataacatccttgagtgtgtctacttggtagatcaaattgttcttctcattgtctaactgtgcattggaaaccatggctttcttgtatttttcttccacttcagacaaagattcctttagttctttaagcccctgcatgtatctcccttctacatcctgtatctggtccttaaggtcatagatatcccgcaattcacttaatgaagtgtctggatctattaagctgctggtgtccccacttcctcgtctggatgagtttccacttagaggggttgttgctgaggcagaatttcgagatgaaggtcttgtataattttcagcatactgtttgtcagatttttcatccaactctttttgttgtcgttccagttctctcatgcgtatatctcttgcttctgcccgggcagcccgttttgctgccagccttgcctctgcctctctggcaatgttactcaaagcttcatcttctgcagaaaatcggtctttcacaggtgttcttttccttccagaagcaggagtccccatcttgtgttcttaatagtcttttaactttgaaagtgatttaactgtgttttcagcccttagtgatggtagctctcctttccactgacatttacatctagaccccttcatttatcttcccacatctgtgttagggcgcgcgctgcgactgcgtcgctgtccgggaagggccgaagagctgctcgcccgcccggcgcccgctggggctatgggcgaggggcgcagctggacgactcagtcctgggtccccggccaggcgggcggggatggacgcggcggctcccggcactggcagccggctagtcggtcaggccgatgtgccctctgcgccgcggctgagacagcgggaaccggccccgggaggagccgcagcctgagcggccgactgaggaggcgaaggatgggcggggccacagggtcgacgac

SEQ ID NO: 16401 - RNA, 2938 nt, Homo sapiens
  source 1..2938: mol_type = other RNA
gtccacttctgcctgccctgccctaccctccccctttgggtttgtttgaggtttcattccacaaataagcagcagataaaatactttacaaggtacagcacagttgtattgaagaaaaaaaggacccaactcttactttaggagtattaggcctggacttcccctgccccatgcaataaagcaagttttatatacactccccatatttttttctaacattttcttatataaatttaaatattttacaaaaaaaggcttttttcctccaaacatataaatctgagtgaaacatagattccccacccgagaacttgtttcttcactaaaatataaatgttgtctgatattaagggtaaatgtcttttgaccactggagatcactgaagtctgaattgcaccgtggagaaggcacttgtgttttctgaggtctccagcaagtatctcagtgagcactcatagaattgctgtctgtcctccagaacccgtgccaaggcctccgagtgcccagttactgaggcagctggggaaaaacgttgagtaaacatgattctacaattacggagataaaaaataaaaacagcatggactggttctaccctagaatcaaactacaacaaaatccaaagtgttcattcatgtagattcaaaatgacttcattctgtcataaattataaaatacaaaggtggctgttttaatgacaaaactcaaaacagtactaaaaggggtttgtgtcaatggacaaaagtcagtccctctaggtagggccccaaggagcatcacccaggttgaagggtggttttcctactgctgggccagaagtgctgtcctattggccttcatcttctccagccgcttggccaggtggctgttggtcatctccatctcctcaatcttgtccagtgctgttcgtaactctcgttgtagcttccgtttttctgctttcaattcatcttcaactttctcagcattctcagcagcagttttatatctcagaacctgtccctcaagccggctaatactttgctccaaggtagttatatcctgttctgcttttgaaagcttaaatttgtattcgctaatttgtctattggcatctctctgcatttcgatgaactgcaagtctgagccattctgcagtcctgccaggtcacccactgtgccatcattcctggagcatttctgtcgttcctcctctaactgaagcttcagttttctaatctgtgacagtagttcttccttctctccagcaagttttcgtagccttacatctaatggcccttctcctgctgactccaagacctgagcagcttcctgagacacaacagtgatggctccagccactggttcatgactgacatcaccattgggagtgccatcggggattataactaagccatgtttctctcccgtcttcactgtctcctgcaggtcagccagctcctctctgagcatatctcgctcattcctaaggcaggcaatgtattctttctgtttctctagggccccaatttttttatctttccaaagaagtgtctcctggaggtcaaacacctcttttgtcatggtgtctattttctgctgcatgcgctgcttctcctcaataagctcatctctttgccgcaggccttctttaagttcttccatcttatgctgcagcacactacacatatgtttctgcctttctaactcctttgatttttcttcattttctctataaaattctgccatctgttcctcctgctcttcaataacatccttgagtgtgtctacttggtagatcaaattgttcttctcattgtctaactgtgcattggaaaccatggctttcttgtatttttcttccacttcagacaaagattcctttagttctttaagcccctgcatgtatctcccttctacatcctgtatctggtccttaaggtcatagatatcccgcaattcacttaatgaagtgtctggatctattaagctgctggtgtccccacttcctcgtctggatgagtttccacttagaggggttgttgctgaggcagaatttcgagatgaaggtcttgtataattttcagcatactgtttgtcagatttttcatccaactctttttgttgtcgttccagttctctcatgcgtatatctcttgcttctgcccgggcagcccgttttgctgccagccttgcctctgcctctctggcaatgttactcaaagcttcatcttctgcagaaaatcggtctttcacaggtgttcttttccttccagaagcaggagtccccatcttgtgttcttaatagtcttttaactttgaaagtgatttaactgtgttttcagcccttagtgatggtagctctcctttccactgacatttacatctagaccccttcatttatcttcccacatcttttccccagcgcggtggaagggtgagcgttagaaatcagacgggatgtctgagaacgccgcaggcagggggcgaccccagcccgggagcccgccgcgggccggccagtccccagggaagcccggccccctagccgaggtcggaggcggcgcggatcccacgggactgcggaggccgggaaaaaggttcccaactccccgctccctgctcccaccgggctggcgggaggagcggcccttacctgtgttagggcgcgcgctgcgactgcgtcgctgtccgggaagggccgaagagctgctcgcccgcccggcgcccgctggggctatgggcgaggggcgcagctggacgactcagtcctgggtccccggccaggcgggcggggatggacgcggcggctcccggcactggcagccggctagtcggtcaggccgatgtgccctctgcgccgcggctgagacagcgggaaccggccccgggaggagccgcagcctgagcggccgactgaggaggcgaaggatgggcggggccacagggtcgacgac

SEQ ID NO: 16402 - RNA, 3356 nt, Homo sapiens
  source 1..3356: mol_type = other RNA
gtccacttctgcctgccctgccctaccctccccctttgggtttgtttgaggtttcattccacaaataagcagcagataaaatactttacaaggtacagcacagttgtattgaagaaaaaaaggacccaactcttactttaggagtattaggcctggacttcccctgccccatgcaataaagcaagttttatatacactccccatatttttttctaacattttcttatataaatttaaatattttacaaaaaaaggcttttttcctccaaacatataaatctgagtgaaacatagattccccacccgagaacttgtttcttcactaaaatataaatgttgtctgatattaagggtaaatgtcttttgaccactggagatcactgaagtctgaattgcaccgtggagaaggcacttgtgttttctgaggtctccagcaagtatctcagtgagcactcatagaattgctgtctgtcctccagaacccgtgccaaggcctccgagtgcccagttactgaggcagctggggaaaaacgttgagtaaacatgattctacaattacggagataaaaaataaaaacagcatggactggttctaccctagaatcaaactacaacaaaatccaaagtgttcattcatgtagattcaaaatgacttcattctgtcataaattataaaatacaaaggtggctgttttaatgacaaaactcaaaacagtactaaaaggggtttgtgtcaatggacaaaagtcagtccctctaggtagggccccaaggagcatcacccaggttgaagggtggttttcctactgctgggccagaagtgctgtcctattggccttcatcttctccagccgcttggccaggtggctgttggtcatctccatctcctcaatcttgtccagtgctgttcgtaactctcgttgtagcttccgtttttctgctttcaattcatcttcaactttctcagcattctcagcagcagttttatatctcagaacctgtccctcaagccggctaatactttgctccaaggtagttatatcctgttctgcttttgaaagcttaaatttgtattcgctaatttgtctattggcatctctctgcatttcgatgaactgcaagtctgagccattctgcagtcctgccaggtcacccactgtgccatcattcctggagcatttctgtcgttcctcctctaactgaagcttcagttttctaatctgtgacagtagttcttccttctctccagcaagttttcgtagccttacatctaatggcccttctcctgctgactccaagacctgagcagcttcctgagacacaacagtgatggctccagccactggttcatgactgacatcaccattgggagtgccatcggggattataactaagccatgtttctctcccgtcttcactgtctcctgcaggtcagccagctcctctctgagcatatctcgctcattcctaaggcaggcaatgtattctttctgtttctctagggccccaatttttttatctttccaaagaagtgtctcctggaggtcaaacacctcttttgtcatggtgtctattttctgctgcatgcgctgcttctcctcaataagctcatctctttgccgcaggccttctttaagttcttccatcttatgctgcagcacactacacatatgtttctgcctttctaactcctttgatttttcttcattttctctataaaattctgccatctgttcctcctgctcttcaataacatccttgagtgtgtctacttggtagatcaaattgttcttctcattgtctaactgtgcattggaaaccatggctttcttgtatttttcttccacttcagacaaagattcctttagttctttaagcccctgcatgtatctcccttctacatcctgtatctggtccttaaggtcatagatatcccgcaattcacttaatgaagtgtctggatctattaagctgctggtgtccccacttcctcgtctggatgagtttccacttagaggggttgttgctgaggcagaatttcgagatgaaggtcttgtataattttcagcatactgtttgtcagatttttcatccaagctggacaaatctgggatactgatatcatccacctcagagacaacacttcccctacgattggagcgactgaaataatcagcggcagataccacactctcccttcgtccacgactggcacgatcagaagacacaatgcttgcagtgtcatcgttggtaaaccctggactgcttcgggctgaacttattcttgatgaataataactgcattcagatggagttcgaggaccataagggttatataatccaccattgtacaatgatgccagactggcacttctcagcagaccagaatttgcagtaggagaggccctgtcactcttatatgttgccagagggtcactgtacagggaagaagaccgagtgtagtaggcagaggtgggtttgctatgtctaagactgctatagtttctctggtcaaagtagaggccactcagtaggtctttatgagaatcagaagacctcttcttcattccatgagagtgactgtaagaatgatttaatgatgaaagtcttgatgatctatccttgaacatatcatacctgtgactgccaacacttcgaatggacaatgcatcctcaactcccagataaggacgatggtgactggaccggtgggaatacctggccctttccgaatcttccagccacttctgaatctgtccccacttccgatcaaaggaatgaagagagtactctttttgttgtcgttccagttctctcatgcgtatatctcttgcttctgcccgggcagcccgttttgctgccagccttgcctctgcctctctggcaatgttactcaaagcttcatcttctgcagaaaatcggtctttcacaggtgttcttttccttccagaagcaggagtccccatcttgtgttcttaatagtcttttaactttgaaagtgatttaactgtgttttcagcccttagtgatggtagctctcctttccactgacatttacatctagaccccttcatttatcttcccacatctgtgttagggcgcgcgctgcgactgcgtcgctgtccgggaagggccgaagagctgctcgcccgcccggcgcccgctggggctatgggcgaggggcgcagctggacgactcagtcctgggtccccggccaggcgggcggggatggacgcggcggctcccggcactggcagccggctagtcggtcaggccgatgtgccctctgcgccgcggctgagacagcgggaaccggccccgggaggagccgcagcctgagcggccgactgaggag

SEQ ID NO: 16403 - RNA, 3317 nt, Homo sapiens
  source 1..3317: mol_type = other RNA
gtccacttctgcctgccctgccctaccctccccctttgggtttgtttgaggtttcattccacaaataagcagcagataaaatactttacaaggtacagcacagttgtattgaagaaaaaaaggacccaactcttactttaggagtattaggcctggacttcccctgccccatgcaataaagcaagttttatatacactccccatatttttttctaacattttcttatataaatttaaatattttacaaaaaaaggcttttttcctccaaacatataaatctgagtgaaacatagattccccacccgagaacttgtttcttcactaaaatataaatgttgtctgatattaagggtaaatgtcttttgaccactggagatcactgaagtctgaattgcaccgtggagaaggcacttgtgttttctgaggtctccagcaagtatctcagtgagcactcatagaattgctgtctgtcctccagaacccgtgccaaggcctccgagtgcccagttactgaggcagctggggaaaaacgttgagtaaacatgattctacaattacggagataaaaaataaaaacagcatggactggttctaccctagaatcaaactacaacaaaatccaaagtgttcattcatgtagattcaaaatgacttcattctgtcataaattataaaatacaaaggtggctgttttaatgacaaaactcaaaacagtactaaaaggggtttgtgtcaatggacaaaagtcagtccctctaggtagggccccaaggagcatcacccaggttgaagggtggttttcctactgctgggccagaagtgctgtcctattggccttcatcttctccagccgcttggccaggtggctgttggtcatctccatctcctcaatcttgtccagtgctgttcgtaactctcgttgtagcttccgtttttctgctttcaattcatcttcaactttctcagcattctcagcagcagttttatatctcagaacctgtccctcaagccggctaatactttgctccaaggtagttatatcctgttctgcttttgaaagcttaaatttgtattcgctaatttgtctattggcatctctctgcatttcgatgaactgcaagtctgagccattctgcagtcctgccaggtcacccactgtgccatcattcctggagcatttctgtcgttcctcctctaactgaagcttcagttttctaatctgtgacagtagttcttccttctctccagcaagttttcgtagccttacatctaatggcccttctcctgctgactccaagacctgagcagcttcctgagacacaacagtgatggctccagccactggttcatgactgacatcaccattgggagtgccatcggggattataactaagccatgtttctctcccgtcttcactgtctcctgcaggtcagccagctcctctctgagcatatctcgctcattcctaaggcaggcaatgtattctttctgtttctctagggccccaatttttttatctttccaaagaagtgtctcctggaggtcaaacacctcttttgtcatggtgtctattttctgctgcatgcgctgcttctcctcaataagctcatctctttgccgcaggccttctttaagttcttccatcttatgctgcagcacactacacatatgtttctgcctttctaactcctttgatttttcttcattttctctataaaattctgccatctgttcctcctgctcttcaataacatccttgagtgtgtctacttggtagatcaaattgttcttctcattgtctaactgtgcattggaaaccatggctttcttgtatttttcttccacttcagacaaagattcctttagttctttaagcccctgcatgtatctcccttctacatcctgtatctggtccttaaggtcatagatatcccgcaattcacttaatgaagtgtctggatctattaagctgctggtgtccccacttcctcgtctggatgagtttccacttagaggggttgttgctgaggcagaatttcgagatgaaggtcttgtataattttcagcatactgtttgtcagatttttcatccaagctggacaaatctgggatactgatatcatccacctcagagacaacacttcccctacgattggagcgactgaaataatcagcggcagataccacactctcccttcgtccacgactggcacgatcagaagacacaatgcttgcagtgtcatcgttggtaaaccctggactgcttcgggctgaacttattcttgatgaataataactgcattcagatggagttcgaggaccataagggttatataatccaccattgtacaatgatgccagactggcacttctcagcagaccagaatttgcagtaggagaggccctgtcactcttatatgttgccagagggtcactgtacagggaagaagactgccgagtgtagtaggcagaggtgggtttgctatgtctaagactgctatagtttctctggtcaaagtagaggccactcagtaggtctttatgagaatcagaagacctcttcttcattccatgagagtgactgtaagaatgattcctgtgactgccaacacttcgaatggacaatgcatcctcaactcccagataaggacgatggtgactggaccggtgggaatacctggccctttccgaatcttccagccacttctgaatctgtccccacttccgatcaaaggaatgaagagagtactctttttgttgtcgttccagttctctcatgcgtatatctcttgcttctgcccgggcagcccgttttgctgccagccttgcctctgcctctctggcaatgttactcaaagcttcatcttctgcagaaaatcggtctttcacaggtgttcttttccttccagaagcaggagtccccatcttgtgttcttaatagtcttttaactttgaaagtgatttaactgtgttttcagcccttagtgatggtagctctcctttccactgacatttacatctagaccccttcatttatcttcccacatctgtgttagggcgcgcgctgcgactgcgtcgctgtccgggaagggccgaagagctgctcgcccgcccggcgcccgctggggctatgggcgaggggcgcagctggacgactcagtcctgggtccccggccaggcgggcggggatggacgcggcggctcccggcactggcagccggctagtcggtcaggccgatgtgccctctgcgccgcggctgagacagcgggaaccggccccgggaggagccgcagcctgagcggccgactgaggag

SEQ ID NO: 16404 - RNA, 3266 nt, Homo sapiens
  source 1..3266: mol_type = other RNA
gtccacttctgcctgccctgccctaccctccccctttgggtttgtttgaggtttcattccacaaataagcagcagataaaatactttacaaggtacagcacagttgtattgaagaaaaaaaggacccaactcttactttaggagtattaggcctggacttcccctgccccatgcaataaagcaagttttatatacactccccatatttttttctaacattttcttatataaatttaaatattttacaaaaaaaggcttttttcctccaaacatataaatctgagtgaaacatagattccccacccgagaacttgtttcttcactaaaatataaatgttgtctgatattaagggtaaatgtcttttgaccactggagatcactgaagtctgaattgcaccgtggagaaggcacttgtgttttctgaggtctccagcaagtatctcagtgagcactcatagaattgctgtctgtcctccagaacccgtgccaaggcctccgagtgcccagttactgaggcagctggggaaaaacgttgagtaaacatgattctacaattacggagataaaaaataaaaacagcatggactggttctaccctagaatcaaactacaacaaaatccaaagtgttcattcatgtagattcaaaatgacttcattctgtcataaattataaaatacaaaggtggctgttttaatgacaaaactcaaaacagtactaaaaggggtttgtgtcaatggacaaaagtcagtccctctaggtagggccccaaggagcatcacccaggttgaagggtggttttcctactgctgggccagaagtgctgtcctattggccttcatcttctccagccgcttggccaggtggctgttggtcatctccatctcctcaatcttgtccagtgctgttcgtaactctcgttgtagcttccgtttttctgctttcaattcatcttcaactttctcagcattctcagcagcagttttatatctcagaacctgtccctcaagccggctaatactttgctccaaggtagttatatcctgttctgcttttgaaagcttaaatttgtattcgctaatttgtctattggcatctctctgcatttcgatgaactgcaagtctgagccattctgcagtcctgccaggtcacccactgtgccatcattcctggagcatttctgtcgttcctcctctaactgaagcttcagttttctaatctgtgacagtagttcttccttctctccagcaagttttcgtagccttacatctaatggcccttctcctgctgactccaagacctgagcagcttcctgagacacaacagtgatggctccagccactggttcatgactgacatcaccattgggagtgccatcggggattataactaagccatgtttctctcccgtcttcactgtctcctgcaggtcagccagctcctctctgagcatatctcgctcattcctaaggcaggcaatgtattctttctgtttctctagggccccaatttttttatctttccaaagaagtgtctcctggaggtcaaacacctcttttgtcatggtgtctattttctgctgcatgcgctgcttctcctcaataagctcatctctttgccgcaggccttctttaagttcttccatcttatgctgcagcacactacacatatgtttctgcctttctaactcctttgatttttcttcattttctctataaaattctgccatctgttcctcctgctcttcaataacatccttgagtgtgtctacttggtagatcaaattgttcttctcattgtctaactgtgcattggaaaccatggctttcttgtatttttcttccacttcagacaaagattcctttagttctttaagcccctgcatgtatctcccttctacatcctgtatctggtccttaaggtcatagatatcccgcaattcacttaatgaagtgtctggatctattaagctgctggtgtccccacttcctcgtctggatgagtttccacttagaggggttgttgctgaggcagaatttcgagatgaaggtcttgtataattttcagcatactgtttgtcagatttttcatccaagctggacaaatctgggatactgatatcatccacctcagagacaacacttcccctacgattggagcgactgaaataatcagcggcagataccacactctcccttcgtccacgactggcacgatcagaagacacaatgcttgcagtgtcatcgttggtaaaccctggactgcttcgggctgaacttattcttgatgaataataactgcattcagatggagttcgaggaccataagggttatataatccaccattgtacaatgatgccagactggcacttctcagcagaccagaatttgcagtaggagaggccctgtcactcttatatgttgccagagggtcactgtacagggaagaagactgccgagtgtagtaggcagaggtgggtttgctatgtctaagactgctatagtttctctggtcaaagtagaggccactcagtaggtctttatgagaatcagaagacctcttcttcattccatgagagtgactgtaagaatgattcctgtgactgccaacacttcgaatggacaatgcatcctcaactcccagataaggacgatggtgactggaccggtgggaatacctggccctttccgaatcttcctctttttgttgtcgttccagttctctcatgcgtatatctcttgcttctgcccgggcagcccgttttgctgccagccttgcctctgcctctctggcaatgttactcaaagcttcatcttctgcagaaaatcggtctttcacaggtgttcttttccttccagaagcaggagtccccatcttgtgttcttaatagtcttttaactttgaaagtgatttaactgtgttttcagcccttagtgatggtagctctcctttccactgacatttacatctagaccccttcatttatcttcccacatctgtgttagggcgcgcgctgcgactgcgtcgctgtccgggaagggccgaagagctgctcgcccgcccggcgcccgctggggctatgggcgaggggcgcagctggacgactcagtcctgggtccccggccaggcgggcggggatggacgcggcggctcccggcactggcagccggctagtcggtcaggccgatgtgccctctgcgccgcggctgagacagcgggaaccggccccgggaggagccgcagcctgagcggccgactgaggag

SEQ ID NO: 16405 - RNA, 3402 nt, Homo sapiens
  source 1..3402: mol_type = other RNA
gtccacttctgcctgccctgccctaccctccccctttgggtttgtttgaggtttcattccacaaataagcagcagataaaatactttacaaggtacagcacagttgtattgaagaaaaaaaggacccaactcttactttaggagtattaggcctggacttcccctgccccatgcaataaagcaagttttatatacactccccatatttttttctaacattttcttatataaatttaaatattttacaaaaaaaggcttttttcctccaaacatataaatctgagtgaaacatagattccccacccgagaacttgtttcttcactaaaatataaatgttgtctgatattaagggtaaatgtcttttgaccactggagatcactgaagtctgaattgcaccgtggagaaggcacttgtgttttctgaggtctccagcaagtatctcagtgagcactcatagaattgctgtctgtcctccagaacccgtgccaaggcctccgagtgcccagttactgaggcagctggggaaaaacgttgagtaaacatgattctacaattacggagataaaaaataaaaacagcatggactggttctaccctagaatcaaactacaacaaaatccaaagtgttcattcatgtagattcaaaatgacttcattctgtcataaattataaaatacaaaggtggctgttttaatgacaaaactcaaaacagtactaaaaggggtttgtgtcaatggacaaaagtcagtccctctaggtagggccccaaggagcatcacccaggttgaagggtggttttcctactgctgggccagaagtgctgtcctattggccttcatcttctccagccgcttggccaggtggctgttggtcatctccatctcctcaatcttgtccagtgctgttcgtaactctcgttgtagcttccgtttttctgctttcaattcatcttcaactttctcagcattctcagcagcagttttatatctcagaacctgtccctcaagccggctaatactttgctccaaggtagttatatcctgttctgcttttgaaagcttaaatttgtattcgctaatttgtctattggcatctctctgcatttcgatgaactgcaagtctgagccattctgcagtcctgccaggtcacccactgtgccatcattcctggagcatttctgtcgttcctcctctaactgaagcttcagttttctaatctgtgacagtagttcttccttctctccagcaagttttcgtagccttacatctaatggcccttctcctgctgactccaagacctgagcagcttcctgagacacaacagtgatggctccagccactggttcatgactgacatcaccattgggagtgccatcggggattataactaagccatgtttctctcccgtcttcactgtctcctgcaggtcagccagctcctctctgagcatatctcgctcattcctaaggcaggcaatgtattctttctgtttctctagggccccaatttttttatctttccaaagaagtgtctcctggaggtcaaacacctcttttgtcatggtgtctattttctgctgcatgcgctgcttctcctcaataagctcatctctttgccgcaggccttctttaagttcttccatcttatgctgcagcacactacacatatgtttctgcctttctaactcctttgatttttcttcattttctctataaaattctgccatctgttcctcctgctcttcaataacatccttgagtgtgtctacttggtagatcaaattgttcttctcattgtctaactgtgcattggaaaccatggctttcttgtatttttcttccacttcagacaaagattcctttagttctttaagcccctgcatgtatctcccttctacatcctgtatctggtccttaaggtcatagatatcccgcaattcacttaatgaagtgtctggatctattaagctgctggtgtccccacttcctcgtctggatgagtttccacttagaggggttgttgctgaggcagaatttcgagatgaaggtcttgtataattttcagcatactgtttgtcagatttttcatccaagctggacaaatctgggatactgatatcatccacctcagagacaacacttcccctacgattggagcgactgaaataatcagcggcagataccacactctcccttcgtccacgactggcacgatcagaagacacaatgcttgcagtgtcatcgttggtaaaccctggactgcttcgggctgaacttattcttgatgaataataactgcattcagatggagttcgaggaccataagggttatataatccaccattgtacaatgatgccagactggcacttctcagcagaccagaatttgcagtaggagaggccctgtcactcttatatgttgccagagggtcactgtacagggaagaagactgccgagtgtagtaggcagaggtgggtttgctatgtctaagactgctatagtttctctggtcaaagtagaggccactcagtaggtctttatgagaatcagaagacctcttcttcattccatgagagtgactgtaagaatgatttaatgatgaaagtcttgatgatctatccttgaacatatcatacctgtgactgccaacacttcgaatggacaatgcatcctcaactcccagataaggacgatggtgactggaccggtgggaatacctggccctttccgaatcttccagccacttctgaatctgtccccacttccgatcaaaggaatgaagagagtactctttttgttgtcgttccagttctctcatgcgtatatctcttgcttctgcccgggcagcccgttttgctgccagccttgcctctgcctctctggcaatgttactcaaagcttcatcttctgcagaaaatcggtctttcacaggtgttcttttccttccagaagcaggagtccccatcttgtgttcttaatagtcttttaactttgaaagtgatttaactgtgttttcagccagaaaagaaggaaagtatcttcaggatcttgcagaatataaaccttagtgatggtagctctcctttccactgacatttacatctagaccccttcatttatcttcccacatctgtgttagggcgcgcgctgcgactgcgtcgctgtccgggaagggccgaagagctgctcgcccgcccggcgcccgctggggctatgggcgaggggcgcagctggacgactcagtcctgggtccccggccaggcgggcggggatggacgcggcggctcccggcactggcagccggctagtcggtcaggccgatgtgccctctgcgccgcggctgagacagcgggaaccggccccgggaggagccgcagcctgagcggccgactgaggag

SEQ ID NO: 16406 - RNA, 3374 nt, Homo sapiens
  source 1..3374: mol_type = other RNA
gtccacttctgcctgccctgccctaccctccccctttgggtttgtttgaggtttcattccacaaataagcagcagataaaatactttacaaggtacagcacagttgtattgaagaaaaaaaggacccaactcttactttaggagtattaggcctggacttcccctgccccatgcaataaagcaagttttatatacactccccatatttttttctaacattttcttatataaatttaaatattttacaaaaaaaggcttttttcctccaaacatataaatctgagtgaaacatagattccccacccgagaacttgtttcttcactaaaatataaatgttgtctgatattaagggtaaatgtcttttgaccactggagatcactgaagtctgaattgcaccgtggagaaggcacttgtgttttctgaggtctccagcaagtatctcagtgagcactcatagaattgctgtctgtcctccagaacccgtgccaaggcctccgagtgcccagttactgaggcagctggggaaaaacgttgagtaaacatgattctacaattacggagataaaaaataaaaacagcatggactggttctaccctagaatcaaactacaacaaaatccaaagtgttcattcatgtagattcaaaatgacttcattctgtcataaattataaaatacaaaggtggctgttttaatgacaaaactcaaaacagtactaaaaggggtttgtgtcaatggacaaaagtcagtccctctaggtagggccccaaggagcatcacccaggttgaagggtggttttcctactgctgggccagaagtgctgtcctattggccttcatcttctccagccgcttggccaggtggctgttggtcatctccatctcctcaatcttgtccagtgctgttcgtaactctcgttgtagcttccgtttttctgctttcaattcatcttcaactttctcagcattctcagcagcagttttatatctcagaacctgtccctcaagccggctaatactttgctccaaggtagttatatcctgttctgcttttgaaagcttaaatttgtattcgctaatttgtctattggcatctctctgcatttcgatgaactgcaagtctgagccattctgcagtcctgccaggtcacccactgtgccatcattcctggagcatttctgtcgttcctcctctaactgaagcttcagttttctaatctgtgacagtagttcttccttctctccagcaagttttcgtagccttacatctaatggcccttctcctgctgactccaagacctgagcagcttcctgagacacaacagtgatggctccagccactggttcatgactgacatcaccattgggagtgccatcggggattataactaagccatgtttctctcccgtcttcactgtctcctgcaggtcagccagctcctctctgagcatatctcgctcattcctaaggcaggcaatgtattctttctgtttctctagggccccaatttttttatctttccaaagaagtgtctcctggaggtcaaacacctcttttgtcatggtgtctattttctgctgcatgcgctgcttctcctcaataagctcatctctttgccgcaggccttctttaagttcttccatcttatgctgcagcacactacacatatgtttctgcctttctaactcctttgatttttcttcattttctctataaaattctgccatctgttcctcctgctcttcaataacatccttgagtgtgtctacttggtagatcaaattgttcttctcattgtctaactgtgcattggaaaccatggctttcttgtatttttcttccacttcagacaaagattcctttagttctttaagcccctgcatgtatctcccttctacatcctgtatctggtccttaaggtcatagatatcccgcaattcacttaatgaagtgtctggatctattaagctgctggtgtccccacttcctcgtctggatgagtttccacttagaggggttgttgctgaggcagaatttcgagatgaaggtcttgtataattttcagcatactgtttgtcagatttttcatccaagctggacaaatctgggatactgatatcatccacctcagagacaacacttcccctacgattggagcgactgaaataatcagcggcagataccacactctcccttcgtccacgactggcacgatcagaagacacaatgcttgcagtgtcatcgttggtaaaccctggactgcttcgggctgaacttattcttgatgaataataactgcattcagatggagttcgaggaccataagggttatataatccaccattgtacaatgatgccagactggcacttctcagcagaccagaatttgcagtaggagaggccctgtcactcttatatgttgccagagggtcactgtacagggaagaagactgccgagtgtagtaggcagaggtgggtttgctatgtctaagactgctatagtttctctggtcaaagtagaggccactcagtaggtctttatgagaatcagaagacctcttcttcattccatgagagtgactgtaagaatgatttaatgatgaaagtcttgatgatctatccttgaacatatcatacctgtgactgccaacacttcgaatggacaatgcatcctcaactcccagataaggacgatggtgactggaccggtgggaatacctggccctttccgaatcttccagccacttctgaatctgtccccacttccgatcaaaggaatgaagagagtactctttttgttgtcgttccagttctctcatgcgtatatctcttgcttctgcccgggcagcccgttttgctgccagccttgcctctgcctctctggcaatgttactcaaagcttcatcttctgcagaaaatcggtctttcacaggtgttcttttccttccagaagcaggagtccccatcttgtgttcttaatagtcttttaactttgaaagtgatttaactgtgttttcagccagaaaagaaggaaagtatcttcaggatcttgcagaatataaaccttagtgatggtagctctcctttccactgacatttacatctagaccccttcatttatcttcccacatcttttccccagcgcggtggaagggtgagcgttagaaatcagacgggatgtctgagaacgccgcaggcagggggcgaccccagcccgggagcccgccgcgggccggccagtccccagggaagcccggccccctagccgaggtcggaggcggcgcggatcccacgggactgcggaggccgggaaaaaggttcccaactccccgctccctgctcccaccgggctggcgggaggagcggccctt

SEQ ID NO: 16407 - RNA, 3470 nt, Homo sapiens
  source 1..3470: mol_type = other RNA
gtccacttctgcctgccctgccctaccctccccctttgggtttgtttgaggtttcattccacaaataagcagcagataaaatactttacaaggtacagcacagttgtattgaagaaaaaaaggacccaactcttactttaggagtattaggcctggacttcccctgccccatgcaataaagcaagttttatatacactccccatatttttttctaacattttcttatataaatttaaatattttacaaaaaaaggcttttttcctccaaacatataaatctgagtgaaacatagattccccacccgagaacttgtttcttcactaaaatataaatgttgtctgatattaagggtaaatgtcttttgaccactggagatcactgaagtctgaattgcaccgtggagaaggcacttgtgttttctgaggtctccagcaagtatctcagtgagcactcatagaattgctgtctgtcctccagaacccgtgccaaggcctccgagtgcccagttactgaggcagctggggaaaaacgttgagtaaacatgattctacaattacggagataaaaaataaaaacagcatggactggttctaccctagaatcaaactacaacaaaatccaaagtgttcattcatgtagattcaaaatgacttcattctgtcataaattataaaatacaaaggtggctgttttaatgacaaaactcaaaacagtactaaaaggggtttgtgtcaatggacaaaagtcagtccctctaggtagggccccaaggagcatcacccaggttgaagggtggttttcctactgctgggccagaagtgctgtcctattggccttcatcttctccagccgcttggccaggtggctgttggtcatctccatctcctcaatcttgtccagtgctgttcgtaactctcgttgtagcttccgtttttctgctttcaattcatcttcaactttctcagcattctcagcagcagttttatatctcagaacctgtccctcaagccggctaatactttgctccaaggtagttatatcctgttctgcttttgaaagcttaaatttgtattcgctaatttgtctattggcatctctctgcatttcgatgaactgcaagtctgagccattctgcagtcctgccaggtcacccactgtgccatcattcctggagcatttctgtcgttcctcctctaactgaagcttcagttttctaatctgtgacagtagttcttccttctctccagcaagttttcgtagccttacatctaatggcccttctcctgctgactccaagacctgagcagcttcctgagacacaacagtgatggctccagccactggttcatgactgacatcaccattgggagtgccatcggggattataactaagccatgtttctctcccgtcttcactgtctcctgcaggtcagccagctcctctctgagcatatctcgctcattcctaaggcaggcaatgtattctttctgtttctctagggccccaatttttttatctttccaaagaagtgtctcctggaggtcaaacacctcttttgtcatggtgtctattttctgctgcatgcgctgcttctcctcaataagctcatctctttgccgcaggccttctttaagttcttccatcttatgctgcagcacactacacatatgtttctgcctttctaactcctttgatttttcttcattttctctataaaattctgccatctgttcctcctgctcttcaataacatccttgagtgtgtctacttggtagatcaaattgttcttctcattgtctaactgtgcattggaaaccatggctttcttgtatttttcttccacttcagacaaagattcctttagttctttaagcccctgcatgtatctcccttctacatcctgtatctggtccttaaggtcatagatatcccgcaattcacttaatgaagtgtctggatctattaagctgctggtgtccccacttcctcgtctggatgagtttccacttagaggggttgttgctgaggcagaatttcgagatgaaggtcttgtataattttcagcatactgtttgtcagatttttcatccaagctggacaaatctgggatactgatatcatccacctcagagacaacacttcccctacgattggagcgactgaaataatcagcggcagataccacactctcccttcgtccacgactggcacgatcagaagacacaatgcttgcagtgtcatcgttggtaaaccctggactgcttcgggctgaacttattcttgatgaataataactgcattcagatggagttcgaggaccataagggttatataatccaccattgtacaatgatgccagactggcacttctcagcagaccagaatttgcagtaggagaggccctgtcactcttatatgttgccagagggtcactgtacagggaagaagactgccgagtgtagtaggcagaggtgggtttgctatgtctaagactgctatagtttctctggtcaaagtagaggccactcagtaggtctttatgagaatcagaagacctcttcttcattccatgagagtgactgtaagaatgatttaatgatgaaagtcttgatgatctatccttgaacatatcatacctgtgactgccaacacttcgaatggacaatgcatcctcaactcccagataaggacgatggtgactggaccggtgggaatacctggccctttccgaatcttccagccacttctgaatctgtccccacttccgatcaaaggaatgaagagagtactctttttgttgtcgttccagttctctcatgcgtatatctcttgcttctgcccgggcagcccgttttgctgccagccttgcctctgcctctctggcaatgttactcaaagcttcatcttctgcagaaaatcggtctttcacaggtgttcttttccttccagaagcaggagtccccatcttgtgttcttaatagtcttttaactttgaaagtgatttaactgtgttttcagccagaaaagaaggaaagtatcttcaggatcttgcagaatataaaccttccaaaacagacagatatttcaataaggctttgtcttctccaatgagcttctcatataatatacgtcttagtgatggtagctctcctttccactgacatttacatctagaccccttcatttatcttcccacatctgtgttagggcgcgcgctgcgactgcgtcgctgtccgggaagggccgaagagctgctcgcccgcccggcgcccgctggggctatgggcgaggggcgcagctggacgactcagtcctgggtccccggccaggcgggcggggatggacgcggcggctcccggcactggcagccggctagtcggtcaggccgatgtgccctctgcgccgcggctgagacagcgggaaccggccccgggaggagccgcagcctgagcggccgactgaggag

SEQ ID NO: 16408 - RNA, 3068 nt, Homo sapiens
  source 1..3068: mol_type = other RNA
gtccacttctgcctgccctgccctaccctccccctttgggtttgtttgaggtttcattccacaaataagcagcagataaaatactttacaaggtacagcacagttgtattgaagaaaaaaaggacccaactcttactttaggagtattaggcctggacttcccctgccccatgcaataaagcaagttttatatacactccccatatttttttctaacattttcttatataaatttaaatattttacaaaaaaaggcttttttcctccaaacatataaatctgagtgaaacatagattccccacccgagaacttgtttcttcactaaaatataaatgttgtctgatattaagggtaaatgtcttttgaccactggagatcactgaagtctgaattgcaccgtggagaaggcacttgtgttttctgaggtctccagcaagtatctcagtgagcactcatagaattgctgtctgtcctccagaacccgtgccaaggcctccgagtgcccagttactgaggcagctggggaaaaacgttgagtaaacatgattctacaattacggagataaaaaataaaaacagcatggactggttctaccctagaatcaaactacaacaaaatccaaagtgttcattcatgtagattcaaaatgacttcattctgtcataaattataaaatacaaaggtggctgttttaatgacaaaactcaaaacagtactaaaaggggtttgtgtcaatggacaaaagtcagtccctctaggtagggccccaaggagcatcacccaggttgaagggtggttttcctactgctgggccagaagtgctgtcctattggccttcatcttctccagccgcttggccaggtggctgttggtcatctccatctcctcaatcttgtccagtgctgttcgtaactctcgttgtagcttccgtttttctgctttcaattcatcttcaactttctcagcattctcagcagcagttttatatctcagaacctgtccctcaagccggctaatactttgctccaaggtagttatatcctgttctgcttttgaaagcttaaatttgtattcgctaatttgtctattggcatctctctgcatttcgatgaactgcaagtctgagccattctgcagtcctgccaggtcacccactgtgccatcattcctggagcatttctgtcgttcctcctctaactgaagcttcagttttctaatctgtgacagtagttcttccttctctccagcaagttttcgtagccttacatctaatggcccttctcctgctgactccaagacctgagcagcttcctgagacacaacagtgatggctccagccactggttcatgactgacatcaccattgggagtgccatcggggattataactaagccatgtttctctcccgtcttcactgtctcctgcaggtcagccagctcctctctgagcatatctcgctcattcctaaggcaggcaatgtattctttctgtttctctagggccccaatttttttatctttccaaagaagtgtctcctggaggtcaaacacctcttttgtcatggtgtctattttctgctgcatgcgctgcttctcctcaataagctcatctctttgccgcaggccttctttaagttcttccatcttatgctgcagcacactacacatatgtttctgcctttctaactcctttgatttttcttcattttctctataaaattctgccatctgttcctcctgctcttcaataacatccttgagtgtgtctacttggtagatcaaattgttcttctcattgtctaactgtgcattggaaaccatggctttcttgtatttttcttccacttcagacaaagattcctttagttctttaagcccctgcatgtatctcccttctacatcctgtatctggtccttaaggtcatagatatcccgcaattcacttaatgaagtgtctggatctattaagctgctggtgtccccacttcctcgtctggatgagtttccacttagaggggttgttgctgaggcagaatttcgagatgaaggtcttgtataattttcagcatactgtttgtcagatttttcatccaagctggacaaatctgggatactgatatcatccacctcagagacaacacttcccctacgattggagcgactgaaataatcagcggcagataccacactctcccttcgtccacgactggcacgatcagaagacacaatgcttgcagtgtcatcgttggtaaaccctggactgcttcgggctgaacttattcttgatgaataataactgcattcagatggagttcgaggaccataagggttatataatccaccattgtacaatgatgccagactggcacttctcagcagaccagaatttgcagtaggagaggccctgtcactcttatatgttgccagagggtcactgtacagggaagaagactgccgagtgtagtaggcagaggtgggtttgctatgtctaagactgctatagtttctctggtcaaagtagaggccactcagtaggtctttatgagaatcagaagacctcttcttcattccatgagagtgactgtaagaatgatttaatgatgaaagtcttgatgatctatccttgaacatatcatacctgtgactgccaacacttcgaatggacaatgcatcctcaactcccagataaggacgatggtgactggaccggtgggaatacctggccctttccgaatcttccagccacttctgaatctgtccccacttccgatcaaaggaatgaagagagtactctttttgttgtcgttccagttctctcatgcgtatatctcttgcttctgcccgggcagcccgttttgctgccagccttgcctctgcctctctggcaatgttactcaaagcttcatcttctgcagaaaatcggtctttcacaggtgttcttttccttccagaagcaggagtccccatcttgtgttcttaatagtcttttaactttgaaagtgatttaactgtgttttcagcccttagtgatggtagctctcctttccactgacatttacatctaga

SEQ ID NO: 16409 - RNA, 3359 nt, Homo sapiens
  source 1..3359: mol_type = other RNA
gtccacttctgcctgccctgccctaccctccccctttgggtttgtttgaggtttcattccacaaataagcagcagataaaatactttacaaggtacagcacagttgtattgaagaaaaaaaggacccaactcttactttaggagtattaggcctggacttcccctgccccatgcaataaagcaagttttatatacactccccatatttttttctaacattttcttatataaatttaaatattttacaaaaaaaggcttttttcctccaaacatataaatctgagtgaaacatagattccccacccgagaacttgtttcttcactaaaatataaatgttgtctgatattaagggtaaatgtcttttgaccactggagatcactgaagtctgaattgcaccgtggagaaggcacttgtgttttctgaggtctccagcaagtatctcagtgagcactcatagaattgctgtctgtcctccagaacccgtgccaaggcctccgagtgcccagttactgaggcagctggggaaaaacgttgagtaaacatgattctacaattacggagataaaaaataaaaacagcatggactggttctaccctagaatcaaactacaacaaaatccaaagtgttcattcatgtagattcaaaatgacttcattctgtcataaattataaaatacaaaggtggctgttttaatgacaaaactcaaaacagtactaaaaggggtttgtgtcaatggacaaaagtcagtccctctaggtagggccccaaggagcatcacccaggttgaagggtggttttcctactgctgggccagaagtgctgtcctattggccttcatcttctccagccgcttggccaggtggctgttggtcatctccatctcctcaatcttgtccagtgctgttcgtaactctcgttgtagcttccgtttttctgctttcaattcatcttcaactttctcagcattctcagcagcagttttatatctcagaacctgtccctcaagccggctaatactttgctccaaggtagttatatcctgttctgcttttgaaagcttaaatttgtattcgctaatttgtctattggcatctctctgcatttcgatgaactgcaagtctgagccattctgcagtcctgccaggtcacccactgtgccatcattcctggagcatttctgtcgttcctcctctaactgaagcttcagttttctaatctgtgacagtagttcttccttctctccagcaagttttcgtagccttacatctaatggcccttctcctgctgactccaagacctgagcagcttcctgagacacaacagtgatggctccagccactggttcatgactgacatcaccattgggagtgccatcggggattataactaagccatgtttctctcccgtcttcactgtctcctgcaggtcagccagctcctctctgagcatatctcgctcattcctaaggcaggcaatgtattctttctgtttctctagggccccaatttttttatctttccaaagaagtgtctcctggaggtcaaacacctcttttgtcatggtgtctattttctgctgcatgcgctgcttctcctcaataagctcatctctttgccgcaggccttctttaagttcttccatcttatgctgcagcacactacacatatgtttctgcctttctaactcctttgatttttcttcattttctctataaaattctgccatctgttcctcctgctcttcaataacatccttgagtgtgtctacttggtagatcaaattgttcttctcattgtctaactgtgcattggaaaccatggctttcttgtatttttcttccacttcagacaaagattcctttagttctttaagcccctgcatgtatctcccttctacatcctgtatctggtccttaaggtcatagatatcccgcaattcacttaatgaagtgtctggatctattaagctgctggtgtccccacttcctcgtctggatgagtttccacttagaggggttgttgctgaggcagaatttcgagatgaaggtcttgtataattttcagcatactgtttgtcagatttttcatccaagctggacaaatctgggatactgatatcatccacctcagagacaacacttcccctacgattggagcgactgaaataatcagcggcagataccacactctcccttcgtccacgactggcacgatcagaagacacaatgcttgcagtgtcatcgttggtaaaccctggactgcttcgggctgaacttattcttgatgaataataactgcattcagatggagttcgaggaccataagggttatataatccaccattgtacaatgatgccagactggcacttctcagcagaccagaatttgcagtaggagaggccctgtcactcttatatgttgccagagggtcactgtacagggaagaagactgccgagtgtagtaggcagaggtgggtttgctatgtctaagactgctatagtttctctggtcaaagtagaggccactcagtaggtctttatgagaatcagaagacctcttcttcattccatgagagtgactgtaagaatgatttaatgatgaaagtcttgatgatctatccttgaacatatcatacctgtgactgccaacacttcgaatggacaatgcatcctcaactcccagataaggacgatggtgactggaccggtgggaatacctggccctttccgaatcttccagccacttctgaatctgtccccacttccgatcaaaggaatgaagagagtactctttttgttgtcgttccagttctctcatgcgtatatctcttgcttctgcccgggcagcccgttttgctgccagccttgcctctgcctctctggcaatgttactcaaagcttcatcttctgcagaaaatcggtctttcacaggtgttcttttccttccagaagcaggagtccccatcttgtgttcttaatagtcttttaactttgaaagtgatttaactgtgttttcagcccttagtgatggtagctctcctttccactgacatttacatctagaccccttcatttatcttcccacatctgtgttagggcgcgcgctgcgactgcgtcgctgtccgggaagggccgaagagctgctcgcccgcccggcgcccgctggggctatgggcgaggggcgcagctggacgactcagtcctgggtccccggccaggcgggcggggatggacgcggcggctcccggcactggcagccggctagtcggtcaggccgatgtgccctctgcgccgcggctgagacagcgggaaccggccccgggaggagccgcagcctgagcggccgactgaggag

SEQ ID NO: 16410 - RNA, 4091 nt, Homo sapiens
  source 1..4091: mol_type = other RNA
gtccacttctgcctgccctgccctaccctccccctttgggtttgtttgaggtttcattccacaaataagcagcagataaaatactttacaaggtacagcacagttgtattgaagaaaaaaaggacccaactcttactttaggagtattaggcctggacttcccctgccccatgcaataaagcaagttttatatacactccccatatttttttctaacattttcttatataaatttaaatattttacaaaaaaaggcttttttcctccaaacatataaatctgagtgaaacatagattccccacccgagaacttgtttcttcactaaaatataaatgttgtctgatattaagggtaaatgtcttttgaccactggagatcactgaagtctgaattgcaccgtggagaaggcacttgtgttttctgaggtctccagcaagtatctcagtgagcactcatagaattgctgtctgtcctccagaacccgtgccaaggcctccgagtgcccagttactgaggcagctggggaaaaacgttgagtaaacatgattctacaattacggagataaaaaataaaaacagcatggactggttctaccctagaatcaaactacaacaaaatccaaagtgttcattcatgtagattcaaaatgacttcattctgtcataaattataaaatacaaaggtggctgttttaatgacaaaactcaaaacagtactaaaaggggtttgtgtcaatggacaaaagtcagtccctctaggtagggccccaaggagcatcacccaggttgaagggtggttttcctactgctgggccagaagtgctgtcctattggccttcatcttctccagccgcttggccaggtggctgttggtcatctccatctcctcaatcttgtccagtgctgttcgtaactctcgttgtagcttccgtttttctgctttcaattcatcttcaactttctcagcattctcagcagcagttttatatctcagaacctgtccctcaagccggctaatactttgctccaaggtagttatatcctgttctgcttttgaaagcttaaatttgtattcgctaatttgtctattggcatctctctgcatttcgatgaactgcaagtctgagccattctgcagtcctgccaggtcacccactgtgccatcattcctggagcatttctgtcgttcctcctctaactgaagcttcagttttctaatctgtgacagtagttcttccttctctccagcaagttttcgtagccttacatctaatggcccttctcctgctgactccaagacctgagcagcttcctgagacacaacagtgatggctccagccactggttcatgactgacatcaccattgggagtgccatcggggattataactaagccatgtttctctcccgtcttcactgtctcctgcaggtcagccagctcctctctgagcatatctcgctcattcctaaggcaggcaatgtattctttctgtttctctagggccccaatttttttatctttccaaagaagtgtctcctggaggtcaaacacctcttttgtcatggtgtctattttctgctgcatgcgctgcttctcctcaataagctcatctctttgccgcaggccttctttaagttcttccatcttatgctgcagcacactacacatatgtttctgcctttctaactcctttgatttttcttcattttctctataaaattctgccatctgttcctcctgctcttcaataacatccttgagtgtgtctacttggtagatcaaattgttcttctcattgtctaactgtgcattggaaaccatggctttcttgtatttttcttccacttcagacaaagattcctttagttctttaagcccctgcatgtatctcccttctacatcctgtatctggtccttaaggtcatagatatcccgcaattcacttaatgaagtgtctggatctattaagctgctggtgtccccacttcctcgtctggatgagtttccacttagaggggttgttgctgaggcagaatttcgagatgaaggtcttgtataattttcagcatactgtttgtcagatttttcatccaagctggacaaatctgggatactgatatcatccacctcagagacaacacttcccctacgattggagcgactgaaataatcagcggcagataccacactctcccttcgtccacgactggcacgatcagaagacacaatgcttgcagtgtcatcgttggtaaaccctggactgcttcgggctgaacttattcttgatgaataataactgcattcagatggagttcgaggaccataagggttatataatccaccattgtacaatgatgccagactggcacttctcagcagaccagaatttgcagtaggagaggccctgtcactcttatatgttgccagagggtcactgtacagggaagaagactgccgagtgtagtaggcagaggtgggtttgctatgtctaagactgctatagtttctctggtcaaagtagaggccactcagtaggtctttatgagaatcagaagacctcttcttcattccatgagagtgactgtaagaatgatttaatgatgaaagtcttgatgatctatccttgaacatatcatacctgtgactgccaacacttcgaatggacaatgcatcctcaactcccagataaggacgatggtgactggaccggtgggaatacctggccctttccgaatcttccagccacttctgaatctgtccccacttccgatcaaaggaatgaagagagtactctttttgttgtcgttccagttctctcatgcgtatatctcttgcttctgcccgggcagcccgttttgctgccagccttgcctctgcctctctggcaatgttactcaaagcttcatcttctgcagaaaatcggtctttcacaggtgttcttttccttccagaagcaggagtccccatcttgtgttcttaatagtcttttaactttgaaagtgatttaactgtgttttcagcccttagtgatggtagctctcctttccactgacatttacatctagaccccttcatttatcttcccacatcttttccccagcgcggtggaagggtgagcgttagaaatcagacgggatgtctgagaacgccgcaggcagggggcgaccccagcccgggagcccgccgcgggccggccagtccccagggaagcccggccccctagccgaggtcggaggcggcgcggatcccacgggactgcggaggccgggaaaaaggttcccaactccccgctccctgctcccaccgggctggcgggaggagcggcccttacctgtgttagggcgcgcgctgcgactgcgtcgctgtccgggaagggccgaagagctgctcgcccgcccggcgcccgctggggctatgggcgaggggcgcagctggacgactcagtcctgggtccccggccaggcgggcggggatggacgcggcggctcccggcactggcagccggctagtcggtcaggccgatgtgccctctgcgccgcggctgagacagcgggaaccggccccgggaggagccgcagcctgagcggccgactgaggaggcgaaggatgggcggggccacagggtcgacgacccactcacccggaagcagttgtggccgcgactgcccgggagtggcgcttgccgcggtccgggcttgcaccccgctgggcaaagtacccggggctgtcacacggcgagctgagccctgggccggcgggtgaggttccccaagcggcgatgcccctggctccctgttccgccattgcgagccgttagggccaagctggagggagggcggcgaggcgcggctgccggtagggcggggccctgggctgctggcggggcggaggccggaggcggccttgggcgggtggcttctctgggtcccacggttcctgcccaggctcttcgaaccaggaccagtgcgggtaatgtgaattgacacttgttccggttcagggctgccccacccctggttgccccaaaccctgcggcctggtgggcttgggcaagtgggctggagtagcgctctgttaggaaacgagtat

SEQ ID NO: 16411 - RNA, 3351 nt, Homo sapiens
  source 1..3351: mol_type = other RNA
gtccacttctgcctgccctgccctaccctccccctttgggtttgtttgaggtttcattccacaaataagcagcagataaaatactttacaaggtacagcacagttgtattgaagaaaaaaaggacccaactcttactttaggagtattaggcctggacttcccctgccccatgcaataaagcaagttttatatacactccccatatttttttctaacattttcttatataaatttaaatattttacaaaaaaaggcttttttcctccaaacatataaatctgagtgaaacatagattccccacccgagaacttgtttcttcactaaaatataaatgttgtctgatattaagggtaaatgtcttttgaccactggagatcactgaagtctgaattgcaccgtggagaaggcacttgtgttttctgaggtctccagcaagtatctcagtgagcactcatagaattgctgtctgtcctccagaacccgtgccaaggcctccgagtgcccagttactgaggcagctggggaaaaacgttgagtaaacatgattctacaattacggagataaaaaataaaaacagcatggactggttctaccctagaatcaaactacaacaaaatccaaagtgttcattcatgtagattcaaaatgacttcattctgtcataaattataaaatacaaaggtggctgttttaatgacaaaactcaaaacagtactaaaaggggtttgtgtcaatggacaaaagtcagtccctctaggtagggccccaaggagcatcacccaggttgaagggtggttttcctactgctgggccagaagtgctgtcctattggccttcatcttctccagccgcttggccaggtggctgttggtcatctccatctcctcaatcttgtccagtgctgttcgtaactctcgttgtagcttccgtttttctgctttcaattcatcttcaactttctcagcattctcagcagcagttttatatctcagaacctgtccctcaagccggctaatactttgctccaaggtagttatatcctgttctgcttttgaaagcttaaatttgtattcgctaatttgtctattggcatctctctgcatttcgatgaactgcaagtctgagccattctgcagtcctgccaggtcacccactgtgccatcattcctggagcatttctgtcgttcctcctctaactgaagcttcagttttctaatctgtgacagtagttcttccttctctccagcaagttttcgtagccttacatctaatggcccttctcctgctgactccaagacctgagcagcttcctgagacacaacagtgatggctccagccactggttcatgactgacatcaccattgggagtgccatcggggattataactaagccatgtttctctcccgtcttcactgtctcctgcaggtcagccagctcctctctgagcatatctcgctcattcctaaggcaggcaatgtattctttctgtttctctagggccccaatttttttatctttccaaagaagtgtctcctggaggtcaaacacctcttttgtcatggtgtctattttctgctgcatgcgctgcttctcctcaataagctcatctctttgccgcaggccttctttaagttcttccatcttatgctgcagcacactacacatatgtttctgcctttctaactcctttgatttttcttcattttctctataaaattctgccatctgttcctcctgctcttcaataacatccttgagtgtgtctacttggtagatcaaattgttcttctcattgtctaactgtgcattggaaaccatggctttcttgtatttttcttccacttcagacaaagattcctttagttctttaagcccctgcatgtatctcccttctacatcctgtatctggtccttaaggtcatagatatcccgcaattcacttaatgaagtgtctggatctattaagctgctggtgtccccacttcctcgtctggatgagtttccacttagaggggttgttgctgaggcagaatttcgagatgaaggtcttgtataattttcagcatactgtttgtcagatttttcatccaagctggacaaatctgggatactgatatcatccacctcagagacaacacttcccctacgattggagcgactgaaataatcagcggcagataccacactctcccttcgtccacgactggcacgatcagaagacacaatgcttgcagtgtcatcgttggtaaaccctggactgcttcgggctgaacttattcttgatgaataataactgcattcagatggagttcgaggaccataagggttatataatccaccattgtacaatgatgccagactggcacttctcagcagaccagaatttgcagtaggagaggccctgtcactcttatatgttgccagagggtcactgtacagggaagaagactgccgagtgtagtaggcagaggtgggtttgctatgtctaagactgctatagtttctctggtcaaagtagaggccactcagtaggtctttatgagaatcagaagacctcttcttcattccatgagagtgactgtaagaatgatttaatgatgaaagtcttgatgatctatccttgaacatatcatacctgtgactgccaacacttcgaatggacaatgcatcctcaactcccagataaggacgatggtgactggaccggtgggaatacctggccctttccgaatcttcctctttttgttgtcgttccagttctctcatgcgtatatctcttgcttctgcccgggcagcccgttttgctgccagccttgcctctgcctctctggcaatgttactcaaagcttcatcttctgcagaaaatcggtctttcacaggtgttcttttccttccagaagcaggagtccccatcttgtgttcttaatagtcttttaactttgaaagtgatttaactgtgttttcagccagaaaagaaggaaagtatcttcaggatcttgcagaatataaaccttagtgatggtagctctcctttccactgacatttacatctagaccccttcatttatcttcccacatctgtgttagggcgcgcgctgcgactgcgtcgctgtccgggaagggccgaagagctgctcgcccgcccggcgcccgctggggctatgggcgaggggcgcagctggacgactcagtcctgggtccccggccaggcgggcggggatggacgcggcggctcccggcactggcagccggctagtcggtcaggccgatgtgccctctgcgccgcggctgagacagcgggaaccggccccgggaggagccgcagcctgagcggccgactgaggag

SEQ ID NO: 16412 - RNA, 3308 nt, Homo sapiens
  source 1..3308: mol_type = other RNA
gtccacttctgcctgccctgccctaccctccccctttgggtttgtttgaggtttcattccacaaataagcagcagataaaatactttacaaggtacagcacagttgtattgaagaaaaaaaggacccaactcttactttaggagtattaggcctggacttcccctgccccatgcaataaagcaagttttatatacactccccatatttttttctaacattttcttatataaatttaaatattttacaaaaaaaggcttttttcctccaaacatataaatctgagtgaaacatagattccccacccgagaacttgtttcttcactaaaatataaatgttgtctgatattaagggtaaatgtcttttgaccactggagatcactgaagtctgaattgcaccgtggagaaggcacttgtgttttctgaggtctccagcaagtatctcagtgagcactcatagaattgctgtctgtcctccagaacccgtgccaaggcctccgagtgcccagttactgaggcagctggggaaaaacgttgagtaaacatgattctacaattacggagataaaaaataaaaacagcatggactggttctaccctagaatcaaactacaacaaaatccaaagtgttcattcatgtagattcaaaatgacttcattctgtcataaattataaaatacaaaggtggctgttttaatgacaaaactcaaaacagtactaaaaggggtttgtgtcaatggacaaaagtcagtccctctaggtagggccccaaggagcatcacccaggttgaagggtggttttcctactgctgggccagaagtgctgtcctattggccttcatcttctccagccgcttggccaggtggctgttggtcatctccatctcctcaatcttgtccagtgctgttcgtaactctcgttgtagcttccgtttttctgctttcaattcatcttcaactttctcagcattctcagcagcagttttatatctcagaacctgtccctcaagccggctaatactttgctccaaggtagttatatcctgttctgcttttgaaagcttaaatttgtattcgctaatttgtctattggcatctctctgcatttcgatgaactgcaagtctgagccattctgcagtcctgccaggtcacccactgtgccatcattcctggagcatttctgtcgttcctcctctaactgaagcttcagttttctaatctgtgacagtagttcttccttctctccagcaagttttcgtagccttacatctaatggcccttctcctgctgactccaagacctgagcagcttcctgagacacaacagtgatggctccagccactggttcatgactgacatcaccattgggagtgccatcggggattataactaagccatgtttctctcccgtcttcactgtctcctgcaggtcagccagctcctctctgagcatatctcgctcattcctaaggcaggcaatgtattctttctgtttctctagggccccaatttttttatctttccaaagaagtgtctcctggaggtcaaacacctcttttgtcatggtgtctattttctgctgcatgcgctgcttctcctcaataagctcatctctttgccgcaggccttctttaagttcttccatcttatgctgcagcacactacacatatgtttctgcctttctaactcctttgatttttcttcattttctctataaaattctgccatctgttcctcctgctcttcaataacatccttgagtgtgtctacttggtagatcaaattgttcttctcattgtctaactgtgcattggaaaccatggctttcttgtatttttcttccacttcagacaaagattcctttagttctttaagcccctgcatgtatctcccttctacatcctgtatctggtccttaaggtcatagatatcccgcaattcacttaatgaagtgtctggatctattaagctgctggtgtccccacttcctcgtctggatgagtttccacttagaggggttgttgctgaggcagaatttcgagatgaaggtcttgtataattttcagcatactgtttgtcagatttttcatccaagctggacaaatctgggatactgatatcatccacctcagagacaacacttcccctacgattggagcgactgaaataatcagcggcagataccacactctcccttcgtccacgactggcacgatcagaagacacaatgcttgcagtgtcatcgttggtaaaccctggactgcttcgggctgaacttattcttgatgaataataactgcattcagatggagttcgaggaccataagggttatataatccaccattgtacaatgatgccagactggcacttctcagcagaccagaatttgcagtaggagaggccctgtcactcttatatgttgccagagggtcactgtacagggaagaagactgccgagtgtagtaggcagaggtgggtttgctatgtctaagactgctatagtttctctggtcaaagtagaggccactcagtaggtctttatgagaatcagaagacctcttcttcattccatgagagtgactgtaagaatgatttaatgatgaaagtcttgatgatctatccttgaacatatcatacctgtgactgccaacacttcgaatggacaatgcatcctcaactcccagataaggacgatggtgactggaccggtgggaatacctggccctttccgaatcttcctctttttgttgtcgttccagttctctcatgcgtatatctcttgcttctgcccgggcagcccgttttgctgccagccttgcctctgcctctctggcaatgttactcaaagcttcatcttctgcagaaaatcggtctttcacaggtgttcttttccttccagaagcaggagtccccatcttgtgttcttaatagtcttttaactttgaaagtgatttaactgtgttttcagcccttagtgatggtagctctcctttccactgacatttacatctagaccccttcatttatcttcccacatctgtgttagggcgcgcgctgcgactgcgtcgctgtccgggaagggccgaagagctgctcgcccgcccggcgcccgctggggctatgggcgaggggcgcagctggacgactcagtcctgggtccccggccaggcgggcggggatggacgcggcggctcccggcactggcagccggctagtcggtcaggccgatgtgccctctgcgccgcggctgagacagcgggaaccggccccgggaggagccgcagcctgagcggccgactgaggag

SEQ ID NO: 16413 - RNA, 4040 nt, Homo sapiens
  source 1..4040: mol_type = other RNA
gtccacttctgcctgccctgccctaccctccccctttgggtttgtttgaggtttcattccacaaataagcagcagataaaatactttacaaggtacagcacagttgtattgaagaaaaaaaggacccaactcttactttaggagtattaggcctggacttcccctgccccatgcaataaagcaagttttatatacactccccatatttttttctaacattttcttatataaatttaaatattttacaaaaaaaggcttttttcctccaaacatataaatctgagtgaaacatagattccccacccgagaacttgtttcttcactaaaatataaatgttgtctgatattaagggtaaatgtcttttgaccactggagatcactgaagtctgaattgcaccgtggagaaggcacttgtgttttctgaggtctccagcaagtatctcagtgagcactcatagaattgctgtctgtcctccagaacccgtgccaaggcctccgagtgcccagttactgaggcagctggggaaaaacgttgagtaaacatgattctacaattacggagataaaaaataaaaacagcatggactggttctaccctagaatcaaactacaacaaaatccaaagtgttcattcatgtagattcaaaatgacttcattctgtcataaattataaaatacaaaggtggctgttttaatgacaaaactcaaaacagtactaaaaggggtttgtgtcaatggacaaaagtcagtccctctaggtagggccccaaggagcatcacccaggttgaagggtggttttcctactgctgggccagaagtgctgtcctattggccttcatcttctccagccgcttggccaggtggctgttggtcatctccatctcctcaatcttgtccagtgctgttcgtaactctcgttgtagcttccgtttttctgctttcaattcatcttcaactttctcagcattctcagcagcagttttatatctcagaacctgtccctcaagccggctaatactttgctccaaggtagttatatcctgttctgcttttgaaagcttaaatttgtattcgctaatttgtctattggcatctctctgcatttcgatgaactgcaagtctgagccattctgcagtcctgccaggtcacccactgtgccatcattcctggagcatttctgtcgttcctcctctaactgaagcttcagttttctaatctgtgacagtagttcttccttctctccagcaagttttcgtagccttacatctaatggcccttctcctgctgactccaagacctgagcagcttcctgagacacaacagtgatggctccagccactggttcatgactgacatcaccattgggagtgccatcggggattataactaagccatgtttctctcccgtcttcactgtctcctgcaggtcagccagctcctctctgagcatatctcgctcattcctaaggcaggcaatgtattctttctgtttctctagggccccaatttttttatctttccaaagaagtgtctcctggaggtcaaacacctcttttgtcatggtgtctattttctgctgcatgcgctgcttctcctcaataagctcatctctttgccgcaggccttctttaagttcttccatcttatgctgcagcacactacacatatgtttctgcctttctaactcctttgatttttcttcattttctctataaaattctgccatctgttcctcctgctcttcaataacatccttgagtgtgtctacttggtagatcaaattgttcttctcattgtctaactgtgcattggaaaccatggctttcttgtatttttcttccacttcagacaaagattcctttagttctttaagcccctgcatgtatctcccttctacatcctgtatctggtccttaaggtcatagatatcccgcaattcacttaatgaagtgtctggatctattaagctgctggtgtccccacttcctcgtctggatgagtttccacttagaggggttgttgctgaggcagaatttcgagatgaaggtcttgtataattttcagcatactgtttgtcagatttttcatccaagctggacaaatctgggatactgatatcatccacctcagagacaacacttcccctacgattggagcgactgaaataatcagcggcagataccacactctcccttcgtccacgactggcacgatcagaagacacaatgcttgcagtgtcatcgttggtaaaccctggactgcttcgggctgaacttattcttgatgaataataactgcattcagatggagttcgaggaccataagggttatataatccaccattgtacaatgatgccagactggcacttctcagcagaccagaatttgcagtaggagaggccctgtcactcttatatgttgccagagggtcactgtacagggaagaagactgccgagtgtagtaggcagaggtgggtttgctatgtctaagactgctatagtttctctggtcaaagtagaggccactcagtaggtctttatgagaatcagaagacctcttcttcattccatgagagtgactgtaagaatgatttaatgatgaaagtcttgatgatctatccttgaacatatcatacctgtgactgccaacacttcgaatggacaatgcatcctcaactcccagataaggacgatggtgactggaccggtgggaatacctggccctttccgaatcttcctctttttgttgtcgttccagttctctcatgcgtatatctcttgcttctgcccgggcagcccgttttgctgccagccttgcctctgcctctctggcaatgttactcaaagcttcatcttctgcagaaaatcggtctttcacaggtgttcttttccttccagaagcaggagtccccatcttgtgttcttaatagtcttttaactttgaaagtgatttaactgtgttttcagcccttagtgatggtagctctcctttccactgacatttacatctagaccccttcatttatcttcccacatcttttccccagcgcggtggaagggtgagcgttagaaatcagacgggatgtctgagaacgccgcaggcagggggcgaccccagcccgggagcccgccgcgggccggccagtccccagggaagcccggccccctagccgaggtcggaggcggcgcggatcccacgggactgcggaggccgggaaaaaggttcccaactccccgctccctgctcccaccgggctggcgggaggagcggcccttacctgtgttagggcgcgcgctgcgactgcgtcgctgtccgggaagggccgaagagctgctcgcccgcccggcgcccgctggggctatgggcgaggggcgcagctggacgactcagtcctgggtccccggccaggcgggcggggatggacgcggcggctcccggcactggcagccggctagtcggtcaggccgatgtgccctctgcgccgcggctgagacagcgggaaccggccccgggaggagccgcagcctgagcggccgactgaggaggcgaaggatgggcggggccacagggtcgacgacccactcacccggaagcagttgtggccgcgactgcccgggagtggcgcttgccgcggtccgggcttgcaccccgctgggcaaagtacccggggctgtcacacggcgagctgagccctgggccggcgggtgaggttccccaagcggcgatgcccctggctccctgttccgccattgcgagccgttagggccaagctggagggagggcggcgaggcgcggctgccggtagggcggggccctgggctgctggcggggcggaggccggaggcggccttgggcgggtggcttctctgggtcccacggttcctgcccaggctcttcgaaccaggaccagtgcgggtaatgtgaattgacacttgttccggttcagggctgccccacccctggttgccccaaaccctgcggcctggtgggcttgggcaagtgggctggagtagcgctctgttaggaaacgagtat

SEQ ID NO: 16414 - RNA, 3251 nt, Homo sapiens
  source 1..3251: mol_type = other RNA
gtccacttctgcctgccctgccctaccctccccctttgggtttgtttgaggtttcattccacaaataagcagcagataaaatactttacaaggtacagcacagttgtattgaagaaaaaaaggacccaactcttactttaggagtattaggcctggacttcccctgccccatgcaataaagcaagttttatatacactccccatatttttttctaacattttcttatataaatttaaatattttacaaaaaaaggcttttttcctccaaacatataaatctgagtgaaacatagattccccacccgagaacttgtttcttcactaaaatataaatgttgtctgatattaagggtaaatgtcttttgaccactggagatcactgaagtctgaattgcaccgtggagaaggcacttgtgttttctgaggtctccagcaagtatctcagtgagcactcatagaattgctgtctgtcctccagaacccgtgccaaggcctccgagtgcccagttactgaggcagctggggaaaaacgttgagtaaacatgattctacaattacggagataaaaaataaaaacagcatggactggttctaccctagaatcaaactacaacaaaatccaaagtgttcattcatgtagattcaaaatgacttcattctgtcataaattataaaatacaaaggtggctgttttaatgacaaaactcaaaacagtactaaaaggggtttgtgtcaatggacaaaagtcagtccctctaggtagggccccaaggagcatcacccaggttgaagggtggttttcctactgctgggccagaagtgctgtcctattggccttcatcttctccagccgcttggccaggtggctgttggtcatctccatctcctcaatcttgtccagtgctgttcgtaactctcgttgtagcttccgtttttctgctttcaattcatcttcaactttctcagcattctcagcagcagttttatatctcagaacctgtccctcaagccggctaatactttgctccaaggtagttatatcctgttctgcttttgaaagcttaaatttgtattcgctaatttgtctattggcatctctctgcatttcgatgaactgcaagtctgagccattctgcagtcctgccaggtcacccactgtgccatcattcctggagcatttctgtcgttcctcctctaactgaagcttcagttttctaatctgtgacagtagttcttccttctctccagcaagttttcgtagccttacatctaatggcccttctcctgctgactccaagacctgagcagcttcctgagacacaacagtgatggctccagccactggttcatgactgacatcaccattgggagtgccatcggggattataactaagccatgtttctctcccgtcttcactgtctcctgcaggtcagccagctcctctctgagcatatctcgctcattcctaaggcaggcaatgtattctttctgtttctctagggccccaatttttttatctttccaaagaagtgtctcctggaggtcaaacacctcttttgtcatggtgtctattttctgctgcatgcgctgcttctcctcaataagctcatctctttgccgcaggccttctttaagttcttccatcttatgctgcagcacactacacatatgtttctgcctttctaactcctttgatttttcttcattttctctataaaattctgccatctgttcctcctgctcttcaataacatccttgagtgtgtctacttggtagatcaaattgttcttctcattgtctaactgtgcattggaaaccatggctttcttgtatttttcttccacttcagacaaagattcctttagttctttaagcccctgcatgtatctcccttctacatcctgtatctggtccttaaggtcatagatatcccgcaattcacttaatgaagtgtctggatctattaagctgctggtgtccccacttcctcgtctggatgagtttccacttagaggggttgttgctgaggcagaatttcgagatgaaggtcttgtataattttcagcatactgtttgtcagatttttcatccaagctggacaaatctgggatactgatatcatccacctcagagacaacacttcccctacgattggagcgactgaaataatcagcggcagataccacactctcccttcgtccacgactggcacgatcagaagacacaatgcttgcagtgtcatcgttggtaaaccctggactgcttcgggctgaacttattcttgatgaataataactgcattcagatggagttcgaggaccataagggttatataatccaccattgtacaatgatgccagactggcacttctcagcagaccagaatttgcagtaggagaggccctgtcactcttatatgttgccagagggtcactgtacagggaagaagactgccgagtgtagtaggcagaggtgggtttgctatgtctaagactgctatagtttctctggtcaaagtagaggccactcagtaggtctttatgagaatcagaagacctcttcttcattccatgagagtgactgtaagaatgatttaatgatgaaagtcttgatgatctatccttgaacatatcatacctgtgactgccaacacttcgaatggacaatgcatcctcaactccctctttttgttgtcgttccagttctctcatgcgtatatctcttgcttctgcccgggcagcccgttttgctgccagccttgcctctgcctctctggcaatgttactcaaagcttcatcttctgcagaaaatcggtctttcacaggtgttcttttccttccagaagcaggagtccccatcttgtgttcttaatagtcttttaactttgaaagtgatttaactgtgttttcagcccttagtgatggtagctctcctttccactgacatttacatctagaccccttcatttatcttcccacatctgtgttagggcgcgcgctgcgactgcgtcgctgtccgggaagggccgaagagctgctcgcccgcccggcgcccgctggggctatgggcgaggggcgcagctggacgactcagtcctgggtccccggccaggcgggcggggatggacgcggcggctcccggcactggcagccggctagtcggtcaggccgatgtgccctctgcgccgcggctgagacagcgggaaccggccccgggaggagccgcagcctgagcggccgactgaggag

SEQ ID NO: 16415 - RNA, 3311 nt, Homo sapiens
  source 1..3311: mol_type = other RNA
gtccacttctgcctgccctgccctaccctccccctttgggtttgtttgaggtttcattccacaaataagcagcagataaaatactttacaaggtacagcacagttgtattgaagaaaaaaaggacccaactcttactttaggagtattaggcctggacttcccctgccccatgcaataaagcaagttttatatacactccccatatttttttctaacattttcttatataaatttaaatattttacaaaaaaaggcttttttcctccaaacatataaatctgagtgaaacatagattccccacccgagaacttgtttcttcactaaaatataaatgttgtctgatattaagggtaaatgtcttttgaccactggagatcactgaagtctgaattgcaccgtggagaaggcacttgtgttttctgaggtctccagcaagtatctcagtgagcactcatagaattgctgtctgtcctccagaacccgtgccaaggcctccgagtgcccagttactgaggcagctggggaaaaacgttgagtaaacatgattctacaattacggagataaaaaataaaaacagcatggactggttctaccctagaatcaaactacaacaaaatccaaagtgttcattcatgtagattcaaaatgacttcattctgtcataaattataaaatacaaaggtggctgttttaatgacaaaactcaaaacagtactaaaaggggtttgtgtcaatggacaaaagtcagtccctctaggtagggccccaaggagcatcacccaggttgaagggtggttttcctactgctgggccagaagtgctgtcctattggccttcatcttctccagccgcttggccaggtggctgttggtcatctccatctcctcaatcttgtccagtgctgttcgtaactctcgttgtagcttccgtttttctgctttcaattcatcttcaactttctcagcattctcagcagcagttttatatctcagaacctgtccctcaagccggctaatactttgctccaaggtagttatatcctgttctgcttttgaaagcttaaatttgtattcgctaatttgtctattggcatctctctgcatttcgatgaactgcaagtctgagccattctgcagtcctgccaggtcacccactgtgccatcattcctggagcatttctgtcgttcctcctctaactgaagcttcagttttctaatctgtgacagtagttcttccttctctccagcaagttttcgtagccttacatctaatggcccttctcctgctgactccaagacctgagcagcttcctgagacacaacagtgatggctccagccactggttcatgactgacatcaccattgggagtgccatcggggattataactaagccatgtttctctcccgtcttcactgtctcctgcaggtcagccagctcctctctgagcatatctcgctcattcctaaggcaggcaatgtattctttctgtttctctagggccccaatttttttatctttccaaagaagtgtctcctggaggtcaaacacctcttttgtcatggtgtctattttctgctgcatgcgctgcttctcctcaataagctcatctctttgccgcaggccttctttaagttcttccatcttatgctgcagcacactacacatatgtttctgcctttctaactcctttgatttttcttcattttctctataaaattctgccatctgttcctcctgctcttcaataacatccttgagtgtgtctacttggtagatcaaattgttcttctcattgtctaactgtgcattggaaaccatggctttcttgtatttttcttccacttcagacaaagattcctttagttctttaagcccctgcatgtatctcccttctacatcctgtatctggtccttaaggtcatagatatcccgcaattcacttaatgaagtgtctggatctattaagctgctggtgtccccacttcctcgtctggatgagtttccacttagaggggttgttgctgaggcagaatttcgagatgaaggtcttgtataattttcagcatactgtttgtcagatttttcatccaagctggacaaatctgggatactgatatcatccacctcagagacaacacttcccctacgattggagcgactgaaataatcagcggcagataccacactctcccttcgtccacgactggcacgatcagaagacacaatgcttgcagtgtcatcgttggtaaaccctggactgcttcgggctgaacttattcttgatgaataataactgcattcagatggagttcgaggaccataagggttatataatccaccattgtacaatgatgccctgtcactcttatatgttgccagagggtcactgtacagggaagaagaccgagtgtagtaggcagaggtgggtttgctatgtctaagactgctatagtttctctggtcaaagtagaggccactcagtaggtctttatgagaatcagaagacctcttcttcattccatgagagtgactgtaagaatgatttaatgatgaaagtcttgatgatctatccttgaacatatcatacctgtgactgccaacacttcgaatggacaatgcatcctcaactcccagataaggacgatggtgactggaccggtgggaatacctggccctttccgaatcttccagccacttctgaatctgtccccacttccgatcaaaggaatgaagagagtactctttttgttgtcgttccagttctctcatgcgtatatctcttgcttctgcccgggcagcccgttttgctgccagccttgcctctgcctctctggcaatgttactcaaagcttcatcttctgcagaaaatcggtctttcacaggtgttcttttccttccagaagcaggagtccccatcttgtgttcttaatagtcttttaactttgaaagtgatttaactgtgttttcagcccttagtgatggtagctctcctttccactgacatttacatctagaccccttcatttatcttcccacatctgtgttagggcgcgcgctgcgactgcgtcgctgtccgggaagggccgaagagctgctcgcccgcccggcgcccgctggggctatgggcgaggggcgcagctggacgactcagtcctgggtccccggccaggcgggcggggatggacgcggcggctcccggcactggcagccggctagtcggtcaggccgatgtgccctctgcgccgcggctgagacagcgggaaccggccccgggaggagccgcagcctgagcggccgactgaggag

SEQ ID NO: 16416 - RNA, 3314 nt, Homo sapiens
  source 1..3314: mol_type = other RNA
gtccacttctgcctgccctgccctaccctccccctttgggtttgtttgaggtttcattccacaaataagcagcagataaaatactttacaaggtacagcacagttgtattgaagaaaaaaaggacccaactcttactttaggagtattaggcctggacttcccctgccccatgcaataaagcaagttttatatacactccccatatttttttctaacattttcttatataaatttaaatattttacaaaaaaaggcttttttcctccaaacatataaatctgagtgaaacatagattccccacccgagaacttgtttcttcactaaaatataaatgttgtctgatattaagggtaaatgtcttttgaccactggagatcactgaagtctgaattgcaccgtggagaaggcacttgtgttttctgaggtctccagcaagtatctcagtgagcactcatagaattgctgtctgtcctccagaacccgtgccaaggcctccgagtgcccagttactgaggcagctggggaaaaacgttgagtaaacatgattctacaattacggagataaaaaataaaaacagcatggactggttctaccctagaatcaaactacaacaaaatccaaagtgttcattcatgtagattcaaaatgacttcattctgtcataaattataaaatacaaaggtggctgttttaatgacaaaactcaaaacagtactaaaaggggtttgtgtcaatggacaaaagtcagtccctctaggtagggccccaaggagcatcacccaggttgaagggtggttttcctactgctgggccagaagtgctgtcctattggccttcatcttctccagccgcttggccaggtggctgttggtcatctccatctcctcaatcttgtccagtgctgttcgtaactctcgttgtagcttccgtttttctgctttcaattcatcttcaactttctcagcattctcagcagcagttttatatctcagaacctgtccctcaagccggctaatactttgctccaaggtagttatatcctgttctgcttttgaaagcttaaatttgtattcgctaatttgtctattggcatctctctgcatttcgatgaactgcaagtctgagccattctgcagtcctgccaggtcacccactgtgccatcattcctggagcatttctgtcgttcctcctctaactgaagcttcagttttctaatctgtgacagtagttcttccttctctccagcaagttttcgtagccttacatctaatggcccttctcctgctgactccaagacctgagcagcttcctgagacacaacagtgatggctccagccactggttcatgactgacatcaccattgggagtgccatcggggattataactaagccatgtttctctcccgtcttcactgtctcctgcaggtcagccagctcctctctgagcatatctcgctcattcctaaggcaggcaatgtattctttctgtttctctagggccccaatttttttatctttccaaagaagtgtctcctggaggtcaaacacctcttttgtcatggtgtctattttctgctgcatgcgctgcttctcctcaataagctcatctctttgccgcaggccttctttaagttcttccatcttatgctgcagcacactacacatatgtttctgcctttctaactcctttgatttttcttcattttctctataaaattctgccatctgttcctcctgctcttcaataacatccttgagtgtgtctacttggtagatcaaattgttcttctcattgtctaactgtgcattggaaaccatggctttcttgtatttttcttccacttcagacaaagattcctttagttctttaagcccctgcatgtatctcccttctacatcctgtatctggtccttaaggtcatagatatcccgcaattcacttaatgaagtgtctggatctattaagctgctggtgtccccacttcctcgtctggatgagtttccacttagaggggttgttgctgaggcagaatttcgagatgaaggtcttgtataattttcagcatactgtttgtcagatttttcatccaagctggacaaatctgggatactgatatcatccacctcagagacaacacttcccctacgattggagcgactgaaataatcagcggcagataccacactctcccttcgtccacgactggcacgatcagaagacacaatgcttgcagtgtcatcgttggtaaaccctggactgcttcgggctgaacttattcttgatgaataataactgcattcagatggagttcgaggaccataagggttatataatccaccattgtacaatgatgccctgtcactcttatatgttgccagagggtcactgtacagggaagaagactgccgagtgtagtaggcagaggtgggtttgctatgtctaagactgctatagtttctctggtcaaagtagaggccactcagtaggtctttatgagaatcagaagacctcttcttcattccatgagagtgactgtaagaatgatttaatgatgaaagtcttgatgatctatccttgaacatatcatacctgtgactgccaacacttcgaatggacaatgcatcctcaactcccagataaggacgatggtgactggaccggtgggaatacctggccctttccgaatcttccagccacttctgaatctgtccccacttccgatcaaaggaatgaagagagtactctttttgttgtcgttccagttctctcatgcgtatatctcttgcttctgcccgggcagcccgttttgctgccagccttgcctctgcctctctggcaatgttactcaaagcttcatcttctgcagaaaatcggtctttcacaggtgttcttttccttccagaagcaggagtccccatcttgtgttcttaatagtcttttaactttgaaagtgatttaactgtgttttcagcccttagtgatggtagctctcctttccactgacatttacatctagaccccttcatttatcttcccacatctgtgttagggcgcgcgctgcgactgcgtcgctgtccgggaagggccgaagagctgctcgcccgcccggcgcccgctggggctatgggcgaggggcgcagctggacgactcagtcctgggtccccggccaggcgggcggggatggacgcggcggctcccggcactggcagccggctagtcggtcaggccgatgtgccctctgcgccgcggctgagacagcgggaaccggccccgggaggagccgcagcctgagcggccgactgaggag

SEQ ID NO: 16417 - RNA, 2600 nt, Homo sapiens
  source 1..2600: mol_type = other RNA
gtccacttctgcctgccctgccctaccctccccctttgggtttgtttgaggtttcattccacaaataagcagcagataaaatactttacaaggtacagcacagttgtattgaagaaaaaaaggacccaactcttactttaggagtattaggcctggacttcccctgccccatgcaataaagcaagttttatatacactccccatatttttttctaacattttcttatataaatttaaatattttacaaaaaaaggcttttttcctccaaacatataaatctgagtgaaacatagattccccacccgagaacttgtttcttcactaaaatataaatgttgtctgatattaagggtaaatgtcttttgaccactggagatcactgaagtctgaattgcaccgtggagaaggcacttgtgttttctgaggtctccagcaagtatctcagtgagcactcatagaattgctgtctgtcctccagaacccgtgccaaggcctccgagtgcccagttactgaggcagctggggaaaaacgttgagtaaacatgattctacaattacggagataaaaaataaaaacagcatggactggttctaccctagaatcaaactacaacaaaatccaaagtgttcattcatgtagattcaaaatgacttcattctgtcataaattataaaatacaaaggtggctgttttaatgacaaaactcaaaacagtactaaaaggggtttgtgtcaatggacaaaagtcagtccctctaggtagggccccaaggagcatcacccaggttgaagggtggttttcctactgctgggccagaagtgctgtcctattggccttcatcttctccagccgcttggccaggtggctgttggtcatctccatctcctcaatcttgtccagtgctgttcgtaactctcgttgtagcttccgtttttctgctttcaattcatcttcaactttctcagcattctcagcagcagttttatatctcagaacctgtccctcaagccggctaatactttgctccaaggtagttatatcctgttctgcttttgaaagcttaaatttgtattcgctaatttgtctattggcatctctctgcatttcgatgaactgcaagtctgagccattctgcagtcctgccaggtcacccactgtgccatcattcctggagcatttctgtcgttcctcctctaactgaagcttcagttttctaatctgtgacagtagttcttccttctctccagcaagttttcgtagccttacatctaatggcccttctcctgctgactccaagacctgagcagcttcctgagacacaacagtgatggctccagccactggttcatgactgacatcaccattgggagtgccatcggggattataactaagccatgtttctctcccgtcttcactgtctcctgcaggtcagccagctcctctctgagcatatctcgctcattcctaaggcaggcaatgtattctttctgtttctctagggcctcaataagctcatctctttgccgcaggccttctttaagttcttccatcttatgctgcagcacactacacatatgtttctgcctttctaactcctttgatttttcttcattttctctataaaattctgccatctgttcctcctgctcttcaataacatccttgagtgtgtctacttggtagatcaaattgttcttctcattgtctaactgtgcattggaaaccatggctttcttgtatttttcttccacttcagacaaagattcccgcaattcacttaatgaagtgtctggatctattaagctgctggtgtccccacttcctcgtctggatgagtttccacttagaggggttgttgctgaggcagaatttcgagatgaaggtcttgtataattttcagcatactgtttgtcagatttttcatccaacctgtgactgccaacacttcgaatggacaatgcatcctcaactcccagataaggacgatggtgactggaccggtgggaatacctggccctttccgaatcttcctctttttgttgtcgttccagttctctcatgcgtatatctcttgcttctgcccgggcagcccgttttgctgccagccttgcctctgcctctctggcaatgttactcaaagcttcatcttctgcagaaaatcggtctttcacaggtgttcttttccttccagaagcaggagtccccatcttgtgttcttaatagtcttttaactttgaaagtgatttaactgtgttttcagcccttagtgatggtagctctcctttccactgacatttacatctagaccccttcatttatcttcccacatctgtgttagggcgcgcgctgcgactgcgtcgctgtccgggaagggccgaagagctgctcgcccgcccggcgcccgctggggctatgggcgaggggcgcagctggacgactcagtcctgggtccccggccaggcgggcggggatggacgcggcggctcccggcactggcagccggctagtcggtcaggccgatgtgccctctgcgccgcggctgagacagcgggaaccggccccgggaggagccgcagcctgagcggccgactgaggag

SEQ ID NO: 16418 - RNA, 2875 nt, Homo sapiens
  source 1..2875: mol_type = other RNA
gtccacttctgcctgccctgccctaccctccccctttgggtttgtttgaggtttcattccacaaataagcagcagataaaatactttacaaggtacagcacagttgtattgaagaaaaaaaggacccaactcttactttaggagtattaggcctggacttcccctgccccatgcaataaagcaagttttatatacactccccatatttttttctaacattttcttatataaatttaaatattttacaaaaaaaggcttttttcctccaaacatataaatctgagtgaaacatagattccccacccgagaacttgtttcttcactaaaatataaatgttgtctgatattaagggtaaatgtcttttgaccactggagatcactgaagtctgaattgcaccgtggagaaggcacttgtgttttctgaggtctccagcaagtatctcagtgagcactcatagaattgctgtctgtcctccagaacccgtgccaaggcctccgagtgcccagttactgaggcagctggggaaaaacgttgagtaaacatgattctacaattacggagataaaaaataaaaacagcatggactggttctaccctagaatcaaactacaacaaaatccaaagtgttcattcatgtagattcaaaatgacttcattctgtcataaattataaaatacaaaggtggctgttttaatgacaaaactcaaaacagtactaaaaggggtttgtgtcaatggacaaaagtcagtccctctaggtagggccccaaggagcatcacccaggttgaagggtggttttcctactgctgggccagaagtgctgtcctattggccttcatcttctccagccgcttggccaggtggctgttggtcatctccatctcctcaatcttgtccagtgctgttcgtaactctcgttgtagcttccgtttttctgctttcaattcatcttcaactttctcagcattctcagcagcagttttatatctcagaacctgtccctcaagccggctaatactttgctccaaggtagttatatcctgttctgcttttgaaagcttaaatttgtattcgctaatttgtctattggcatctctctgcatttcgatgaactgcaagtctgagccattctgcagtcctgccaggtcacccactgtgccatcattcctggagcatttctgtcgttcctcctctaactgaagcttcagttttctaatctgtgacagtagttcttccttctctccagcaagttttcgtagccttacatctaatggcccttctcctgctgactccaagacctgagcagcttcctgagacacaacagtgatggctccagccactggttcatgactgacatcaccattgggagtgccatcggggattataactaagccatgtttctctcccgtcttcactgtctcctgcaggtcagccagctcctctctgagcatatctcgctcattcctaaggcaggcaatgtattctttctgtttctctagggcctcaataagctcatctctttgccgcaggccttctttaagttcttccatcttatgctgcagcacactacacatatgtttctgcctttctaactcctttgatttttcttcattttctctataaaattctgccatctgttcctcctgctcttcaataacatccttgagtgtgtctacttggtagatcaaattgttcttctcattgtctaactgtgcattggaaaccatggctttcttgtatttttcttccacttcagacaaagattcccgcaattcacttaatgaagtgtctggatctattaagctgctggtgtccccacttcctcgtctggatgagtttccacttagaggggttgttgctgaggcagaatttcgagatgaaggtcttgtataattttcagcatactgtttgtcagatttttcatccaacctgtgactgccaacacttcgaatggacaatgcatcctcaactcccagataaggacgatggtgactggaccggtgggaatacctggccctttccgaatcttcctctttttgttgtcgttccagttctctcatgcgtatatctcttgcttctgcccgggcagcccgttttgctgccagccttgcctctgcctctctggcaatgttactcaaagcttcatcttctgcagaaaatcggtctttcacaggtgttcttttccttccagaagcaggagtccccatcttgtgttcttaatagtcttttaactttgaaagtgatttaactgtgttttcagcccttagtgatggtagctctcctttccactgacatttacatctagaccccttcatttatcttcccacatcttttccccagcgcggtggaagggtgagcgttagaaatcagacgggatgtctgagaacgccgcaggcagggggcgaccccagcccgggagcccgccgcgggccggccagtccccagggaagcccggccccctagccgaggtcggaggcggcgcggatcccacgggactgcggaggccgggaaaaaggttcccaactccccgctccctgctcccaccgggctggcgggaggagcggcccttacctgtgttagggcgcgcgctgcgactgcgtcgctgtccgggaagggccgaagagctgctcgcccgcccggcgcccgctggggctatgggcgaggggcgcagctggacgactcagtcctgggtccccggccaggcgggcggggatggacgcggcggctcccggcactggcagccggctagtcggtcaggccgatgtgccctctgcgccgcggctgagacagcgggaaccggccccgggaggagccgcagcctgagcggccgactgaggaggcgaaggatgggcggggccacagggtcgacgac

SEQ ID NO: 16419 - RNA, 2531 nt, Homo sapiens
  source 1..2531: mol_type = other RNA
gtccacttctgcctgccctgccctaccctccccctttgggtttgtttgaggtttcattccacaaataagcagcagataaaatactttacaaggtacagcacagttgtattgaagaaaaaaaggacccaactcttactttaggagtattaggcctggacttcccctgccccatgcaataaagcaagttttatatacactccccatatttttttctaacattttcttatataaatttaaatattttacaaaaaaaggcttttttcctccaaacatataaatctgagtgaaacatagattccccacccgagaacttgtttcttcactaaaatataaatgttgtctgatattaagggtaaatgtcttttgaccactggagatcactgaagtctgaattgcaccgtggagaaggcacttgtgttttctgaggtctccagcaagtatctcagtgagcactcatagaattgctgtctgtcctccagaacccgtgccaaggcctccgagtgcccagttactgaggcagctggggaaaaacgttgagtaaacatgattctacaattacggagataaaaaataaaaacagcatggactggttctaccctagaatcaaactacaacaaaatccaaagtgttcattcatgtagattcaaaatgacttcattctgtcataaattataaaatacaaaggtggctgttttaatgacaaaactcaaaacagtactaaaaggggtttgtgtcaatggacaaaagtcagtccctctaggtagggccccaaggagcatcacccaggttgaagggtggttttcctactgctgggccagaagtgctgtcctattggccttcatcttctccagccgcttggccaggtggctgttggtcatctccatctcctcaatcttgtccagtgctgttcgtaactctcgttgtagcttccgtttttctgctttcaattcatcttcaactttctcagcattctcagcagcagttttatatctcagaacctgtccctcaagccggctaatactttgctccaaggtagttatatcctgttctgcttttgaaagcttaaatttgtattcgctaatttgtctattggcatctctctgcatttcgatgaactgcaagtctgagccattctgcagtcctgccaggtcacccactgtgccatcattcctggagcatttctgtcgttcctcctctaactgaagcttcagttttctaatctgtgacagtagttcttccttctctccagcaagttttcgtagccttacatctaatggcccttctcctgctgactccaagacctgagcagcttcctgagacacaacagtgatggctccagccactggttcatgactgacatcaccattgggagtgccatcggggattataactaagccatgtttctctcccgtcttcactgtctcctgcaggtcagccagctcctctctgagcatatctcgctcattcctaaggcaggcaatgtattctttctgtttctctagggcctcaataagctcatctctttgccgcaggccttctttaagttcttccatcttatgctgcagcacactacacatatgtttctgcctttctaactcctttgatttttcttcattttctctataaaattctgccatctgttcctcctgctcttcaataacatccttgagtgtgtctacttggtagatcaaattgttcttctcattgtctaactgtgcattggaaaccatggctttcttgtatttttcttccacttcagacaaagattcccgcaattcacttaatgaagtgtctggatctattaagctgctggtgtccccacttcctcgtctggatgagtttccacttagaggggttgttgctgaggcagaatttcgagatgaaggtcttgtataattttcagcatactgtttgtcagatttttcatccaactctttttgttgtcgttccagttctctcatgcgtatatctcttgcttctgcccgggcagcccgttttgctgccagccttgcctctgcctctctggcaatgttactcaaagcttcatcttctgcagaaaatcggtctttcacaggtgttcttttccttccagaagcaggagtccccatcttgtgttcttaatagtcttttaactttgaaagtgatttaactgtgttttcagcccttagtgatggtagctctcctttccactgacatttacatctagaccccttcatttatcttcccacatctgtgttagggcgcgcgctgcgactgcgtcgctgtccgggaagggccgaagagctgctcgcccgcccggcgcccgctggggctatgggcgaggggcgcagctggacgactcagtcctgggtccccggccaggcgggcggggatggacgcggcggctcccggcactggcagccggctagtcggtcaggccgatgtgccctctgcgccgcggctgagacagcgggaaccggccccgggaggagccgcagcctgagcggccgactgaggaggcgaaggatgggcggggccacagggtcgacgac

SEQ ID NO: 16420 - RNA, 2773 nt, Homo sapiens
  source 1..2773: mol_type = other RNA
gtccacttctgcctgccctgccctaccctccccctttgggtttgtttgaggtttcattccacaaataagcagcagataaaatactttacaaggtacagcacagttgtattgaagaaaaaaaggacccaactcttactttaggagtattaggcctggacttcccctgccccatgcaataaagcaagttttatatacactccccatatttttttctaacattttcttatataaatttaaatattttacaaaaaaaggcttttttcctccaaacatataaatctgagtgaaacatagattccccacccgagaacttgtttcttcactaaaatataaatgttgtctgatattaagggtaaatgtcttttgaccactggagatcactgaagtctgaattgcaccgtggagaaggcacttgtgttttctgaggtctccagcaagtatctcagtgagcactcatagaattgctgtctgtcctccagaacccgtgccaaggcctccgagtgcccagttactgaggcagctggggaaaaacgttgagtaaacatgattctacaattacggagataaaaaataaaaacagcatggactggttctaccctagaatcaaactacaacaaaatccaaagtgttcattcatgtagattcaaaatgacttcattctgtcataaattataaaatacaaaggtggctgttttaatgacaaaactcaaaacagtactaaaaggggtttgtgtcaatggacaaaagtcagtccctctaggtagggccccaaggagcatcacccaggttgaagggtggttttcctactgctgggccagaagtgctgtcctattggccttcatcttctccagccgcttggccaggtggctgttggtcatctccatctcctcaatcttgtccagtgctgttcgtaactctcgttgtagcttccgtttttctgctttcaattcatcttcaactttctcagcattctcagcagcagttttatatctcagaacctgtccctcaagccggctaatactttgctccaaggtagttatatcctgttctgcttttgaaagcttaaatttgtattcgctaatttgtctattggcatctctctgcatttcgatgaactgcaagtctgagccattctgcagtcctgccaggtcacccactgtgccatcattcctggagcatttctgtcgttcctcctctaactgaagcttcagttttctaatctgtgacagtagttcttccttctctccagcaagttttcgtagccttacatctaatggcccttctcctgctgactccaagacctgagcagcttcctgagacacaacagtgatggctccagccactggttcatgactgacatcaccattgggagtgccatcggggattataactaagccatgtttctctcccgtcttcactgtctcctgcaggtcagccagctcctctctgagcatatctcgctcattcctaaggcaggcaatgtattctttctgtttctctagggcctcaataagctcatctctttgccgcaggccttctttaagttcttccatcttatgctgcagcacactacacatatgtttctgcctttctaactcctttgatttttcttcattttctctataaaattctgccatctgttcctcctgctcttcaataacatccttgagtgtgtctacttggtagatcaaattgttcttctcattgtctaactgtgcattggaaaccatggctttcttgtatttttcttccacttcagacaaagattcccgcaattcacttaatgaagtgtctggatctattaagctgctggtgtccccacttcctcgtctggatgagtttccacttagaggggttgttgctgaggcagaatttcgagatgaaggtcttgtataattttcagcatactgtttgtcagatttttcatccaactctttttgttgtcgttccagttctctcatgcgtatatctcttgcttctgcccgggcagcccgttttgctgccagccttgcctctgcctctctggcaatgttactcaaagcttcatcttctgcagaaaatcggtctttcacaggtgttcttttccttccagaagcaggagtccccatcttgtgttcttaatagtcttttaactttgaaagtgatttaactgtgttttcagcccttagtgatggtagctctcctttccactgacatttacatctagaccccttcatttatcttcccacatcttttccccagcgcggtggaagggtgagcgttagaaatcagacgggatgtctgagaacgccgcaggcagggggcgaccccagcccgggagcccgccgcgggccggccagtccccagggaagcccggccccctagccgaggtcggaggcggcgcggatcccacgggactgcggaggccgggaaaaaggttcccaactccccgctccctgctcccaccgggctggcgggaggagcggcccttacctgtgttagggcgcgcgctgcgactgcgtcgctgtccgggaagggccgaagagctgctcgcccgcccggcgcccgctggggctatgggcgaggggcgcagctggacgactcagtcctgggtccccggccaggcgggcggggatggacgcggcggctcccggcactggcagccggctagtcggtcaggccgatgtgccctctgcgccgcggctgagacagcgggaaccggccccgggaggagccgcagcctgagcggccgactgaggaggcgaaggatgggcggggccacagggtcgacgac

SEQ ID NO: 16421 - RNA, 3194 nt, Homo sapiens
  source 1..3194: mol_type = other RNA
gtccacttctgcctgccctgccctaccctccccctttgggtttgtttgaggtttcattccacaaataagcagcagataaaatactttacaaggtacagcacagttgtattgaagaaaaaaaggacccaactcttactttaggagtattaggcctggacttcccctgccccatgcaataaagcaagttttatatacactccccatatttttttctaacattttcttatataaatttaaatattttacaaaaaaaggcttttttcctccaaacatataaatctgagtgaaacatagattccccacccgagaacttgtttcttcactaaaatataaatgttgtctgatattaagggtaaatgtcttttgaccactggagatcactgaagtctgaattgcaccgtggagaaggcacttgtgttttctgaggtctccagcaagtatctcagtgagcactcatagaattgctgtctgtcctccagaacccgtgccaaggcctccgagtgcccagttactgaggcagctggggaaaaacgttgagtaaacatgattctacaattacggagataaaaaataaaaacagcatggactggttctaccctagaatcaaactacaacaaaatccaaagtgttcattcatgtagattcaaaatgacttcattctgtcataaattataaaatacaaaggtggctgttttaatgacaaaactcaaaacagtactaaaaggggtttgtgtcaatggacaaaagtcagtccctctaggtagggccccaaggagcatcacccaggttgaagggtggttttcctactgctgggccagaagtgctgtcctattggccttcatcttctccagccgcttggccaggtggctgttggtcatctccatctcctcaatcttgtccagtgctgttcgtaactctcgttgtagcttccgtttttctgctttcaattcatcttcaactttctcagcattctcagcagcagttttatatctcagaacctgtccctcaagccggctaatactttgctccaaggtagttatatcctgttctgcttttgaaagcttaaatttgtattcgctaatttgtctattggcatctctctgcatttcgatgaactgcaagtctgagccattctgcagtcctgccaggtcacccactgtgccatcattcctggagcatttctgtcgttcctcctctaactgaagcttcagttttctaatctgtgacagtagttcttccttctctccagcaagttttcgtagccttacatctaatggcccttctcctgctgactccaagacctgagcagcttcctgagacacaacagtgatggctccagccactggttcatgactgacatcaccattgggagtgccatcggggattataactaagccatgtttctctcccgtcttcactgtctcctgcaggtcagccagctcctctctgagcatatctcgctcattcctaaggcaggcaatgtattctttctgtttctctagggcctcaataagctcatctctttgccgcaggccttctttaagttcttccatcttatgctgcagcacactacacatatgtttctgcctttctaactcctttgatttttcttcattttctctataaaattctgccatctgttcctcctgctcttcaataacatccttgagtgtgtctacttggtagatcaaattgttcttctcattgtctaactgtgcattggaaaccatggctttcttgtatttttcttccacttcagacaaagattcccgcaattcacttaatgaagtgtctggatctattaagctgctggtgtccccacttcctcgtctggatgagtttccacttagaggggttgttgctgaggcagaatttcgagatgaaggtcttgtataattttcagcatactgtttgtcagatttttcatccaagctggacaaatctgggatactgatatcatccacctcagagacaacacttcccctacgattggagcgactgaaataatcagcggcagataccacactctcccttcgtccacgactggcacgatcagaagacacaatgcttgcagtgtcatcgttggtaaaccctggactgcttcgggctgaacttattcttgatgaataataactgcattcagatggagttcgaggaccataagggttatataatccaccattgtacaatgatgccagactggcacttctcagcagaccagaatttgcagtaggagaggccctgtcactcttatatgttgccagagggtcactgtacagggaagaagactgccgagtgtagtaggcagaggtgggtttgctatgtctaagactgctatagtttctctggtcaaagtagaggccactcagtaggtctttatgagaatcagaagacctcttcttcattccatgagagtgactgtaagaatgatttaatgatgaaagtcttgatgatctatccttgaacatatcatacctgtgactgccaacacttcgaatggacaatgcatcctcaactcccagataaggacgatggtgactggaccggtgggaatacctggccctttccgaatcttccagccacttctgaatctgtccccacttccgatcaaaggaatgaagagagtactctttttgttgtcgttccagttctctcatgcgtatatctcttgcttctgcccgggcagcccgttttgctgccagccttgcctctgcctctctggcaatgttactcaaagcttcatcttctgcagaaaatcggtctttcacaggtgttcttttccttccagaagcaggagtccccatcttgtgttcttaatagtcttttaactttgaaagtgatttaactgtgttttcagcccttagtgatggtagctctcctttccactgacatttacatctagaccccttcatttatcttcccacatctgtgttagggcgcgcgctgcgactgcgtcgctgtccgggaagggccgaagagctgctcgcccgcccggcgcccgctggggctatgggcgaggggcgcagctggacgactcagtcctgggtccccggccaggcgggcggggatggacgcggcggctcccggcactggcagccggctagtcggtcaggccgatgtgccctctgcgccgcggctgagacagcgggaaccggccccgggaggagccgcagcctgagcggccgactgaggag

SEQ ID NO: 16422 - RNA, 3089 nt, Homo sapiens
  source 1..3089: mol_type = other RNA
gtccacttctgcctgccctgccctaccctccccctttgggtttgtttgaggtttcattccacaaataagcagcagataaaatactttacaaggtacagcacagttgtattgaagaaaaaaaggacccaactcttactttaggagtattaggcctggacttcccctgccccatgcaataaagcaagttttatatacactccccatatttttttctaacattttcttatataaatttaaatattttacaaaaaaaggcttttttcctccaaacatataaatctgagtgaaacatagattccccacccgagaacttgtttcttcactaaaatataaatgttgtctgatattaagggtaaatgtcttttgaccactggagatcactgaagtctgaattgcaccgtggagaaggcacttgtgttttctgaggtctccagcaagtatctcagtgagcactcatagaattgctgtctgtcctccagaacccgtgccaaggcctccgagtgcccagttactgaggcagctggggaaaaacgttgagtaaacatgattctacaattacggagataaaaaataaaaacagcatggactggttctaccctagaatcaaactacaacaaaatccaaagtgttcattcatgtagattcaaaatgacttcattctgtcataaattataaaatacaaaggtggctgttttaatgacaaaactcaaaacagtactaaaaggggtttgtgtcaatggacaaaagtcagtccctctaggtagggccccaaggagcatcacccaggttgaagggtggttttcctactgctgggccagaagtgctgtcctattggccttcatcttctccagccgcttggccaggtggctgttggtcatctccatctcctcaatcttgtccagtgctgttcgtaactctcgttgtagcttccgtttttctgctttcaattcatcttcaactttctcagcattctcagcagcagttttatatctcagaacctgtccctcaagccggctaatactttgctccaaggtagttatatcctgttctgcttttgaaagcttaaatttgtattcgctaatttgtctattggcatctctctgcatttcgatgaactgcaagtctgagccattctgcagtcctgccaggtcacccactgtgccatcattcctggagcatttctgtcgttcctcctctaactgaagcttcagttttctaatctgtgacagtagttcttccttctctccagcaagttttcgtagccttacatctaatggcccttctcctgctgactccaagacctgagcagcttcctgagacacaacagtgatggctccagccactggttcatgactgacatcaccattgggagtgccatcggggattataactaagccatgtttctctcccgtcttcactgtctcctgcaggtcagccagctcctctctgagcatatctcgctcattcctaaggcaggcaatgtattctttctgtttctctagggcctcaataagctcatctctttgccgcaggccttctttaagttcttccatcttatgctgcagcacactacacatatgtttctgcctttctaactcctttgatttttcttcattttctctataaaattctgccatctgttcctcctgctcttcaataacatccttgagtgtgtctacttggtagatcaaattgttcttctcattgtctaactgtgcattggaaaccatggctttcttgtatttttcttccacttcagacaaagattcccgcaattcacttaatgaagtgtctggatctattaagctgctggtgtccccacttcctcgtctggatgagtttccacttagaggggttgttgctgaggcagaatttcgagatgaaggtcttgtataattttcagcatactgtttgtcagatttttcatccaagctggacaaatctgggatactgatatcatccacctcagagacaacacttcccctacgattggagcgactgaaataatcagcggcagataccacactctcccttcgtccacgactggcacgatcagaagacacaatgcttgcagtgtcatcgttggtaaaccctggactgcttcgggctgaacttattcttgatgaataataactgcattcagatggagttcgaggaccataagggttatataatccaccattgtacaatgatgccctgtcactcttatatgttgccagagggtcactgtacagggaagaagactgccgagtgtagtaggcagaggtgggtttgctatgtctaagactgctatagtttctctggtcaaagtagaggccactcagtaggtctttatgagaatcagaagacctcttcttcattccatgagagtgactgtaagaatgattcctgtgactgccaacacttcgaatggacaatgcatcctcaactcccagataaggacgatggtgactggaccggtgggaatacctggccctttccgaatcttcctctttttgttgtcgttccagttctctcatgcgtatatctcttgcttctgcccgggcagcccgttttgctgccagccttgcctctgcctctctggcaatgttactcaaagcttcatcttctgcagaaaatcggtctttcacaggtgttcttttccttccagaagcaggagtccccatcttgtgttcttaatagtcttttaactttgaaagtgatttaactgtgttttcagcccttagtgatggtagctctcctttccactgacatttacatctagaccccttcatttatcttcccacatctgtgttagggcgcgcgctgcgactgcgtcgctgtccgggaagggccgaagagctgctcgcccgcccggcgcccgctggggctatgggcgaggggcgcagctggacgactcagtcctgggtccccggccaggcgggcggggatggacgcggcggctcccggcactggcagccggctagtcggtcaggccgatgtgccctctgcgccgcggctgagacagcgggaaccggccccgggaggagccgcagcctgagcggccgactgaggaggcgaaggatgggcggggccacagggtcgacgac

SEQ ID NO: 16423 - RNA, 2990 nt, Homo sapiens
  source 1..2990: mol_type = other RNA
gtccacttctgcctgccctgccctaccctccccctttgggtttgtttgaggtttcattccacaaataagcagcagataaaatactttacaaggtacagcacagttgtattgaagaaaaaaaggacccaactcttactttaggagtattaggcctggacttcccctgccccatgcaataaagcaagttttatatacactccccatatttttttctaacattttcttatataaatttaaatattttacaaaaaaaggcttttttcctccaaacatataaatctgagtgaaacatagattccccacccgagaacttgtttcttcactaaaatataaatgttgtctgatattaagggtaaatgtcttttgaccactggagatcactgaagtctgaattgcaccgtggagaaggcacttgtgttttctgaggtctccagcaagtatctcagtgagcactcatagaattgctgtctgtcctccagaacccgtgccaaggcctccgagtgcccagttactgaggcagctggggaaaaacgttgagtaaacatgattctacaattacggagataaaaaataaaaacagcatggactggttctaccctagaatcaaactacaacaaaatccaaagtgttcattcatgtagattcaaaatgacttcattctgtcataaattataaaatacaaaggtggctgttttaatgacaaaactcaaaacagtactaaaaggggtttgtgtcaatggacaaaagtcagtccctctaggtagggccccaaggagcatcacccaggttgaagggtggttttcctactgctgggccagaagtgctgtcctattggccttcatcttctccagccgcttggccaggtggctgttggtcatctccatctcctcaatcttgtccagtgctgttcgtaactctcgttgtagcttccgtttttctgctttcaattcatcttcaactttctcagcattctcagcagcagttttatatctcagaacctgtccctcaagccggctaatactttgctccaaggtagttatatcctgttctgcttttgaaagcttaaatttgtattcgctaatttgtctattggcatctctctgcatttcgatgaactgcaagtctgagccattctgcagtcctgccaggtcacccactgtgccatcattcctggagcatttctgtcgttcctcctctaactgaagcttcagttttctaatctgtgacagtagttcttccttctctccagcaagttttcgtagccttacatctaatggcccttctcctgctgactccaagacctgagcagcttcctgagacacaacagtgatggctccagccactggttcatgactgacatcaccattgggagtgccatcggggattataactaagccatgtttctctcccgtcttcactgtctcctgcaggtcagccagctcctctctgagcatatctcgctcattcctaaggcaggcaatgtattctttctgtttctctagggcctcaataagctcatctctttgccgcaggccttctttaagttcttccatcttatgctgcagcacactacacatatgtttctgcctttctaactcctttgatttttcttcattttctctataaaattctgccatctgttcctcctgctcttcaataacatccttgagtgtgtctacttggtagatcaaattgttcttctcattgtctaactgtgcattggaaaccatggctttcttgtatttttcttccacttcagacaaagattcctttagttctttaagcccctgcatgtatctcccttctacatcctgtatctggtccttaaggtcatagatatcccgcaattcacttaatgaagtgtctggatctattaagctgctggtgtccccacttcctcgtctggatgagtttccacttagaggggttgttgctgaggcagaatttcgagatgaaggtcttgtataattttcagcatactgtttgtcagatttttcatccaacacactctcccttcgtccacgactggcacgatcagaagacacaatgcttgcagtgtcatcgttggtaaaccctggactgcttcgggctgaacttattcttgatgaataataactgcattcagatggagttcgaggaccataagggttatataatccaccattgtacaatgatgccctgtgactgccaacacttcgaatggacaatgcatcctcaactcccagataaggacgatggtgactggaccggtgggaatacctggccctttccgaatcttcctctttttgttgtcgttccagttctctcatgcgtatatctcttgcttctgcccgggcagcccgttttgctgccagccttgcctctgcctctctggcaatgttactcaaagcttcatcttctgcagaaaatcggtctttcacaggtgttcttttccttccagaagcaggagtccccatcttgtgttcttaatagtcttttaactttgaaagtgatttaactgtgttttcagccagaaaagaaggaaagtatcttcaggatcttgcagaatataaaccttccaaaacagacagatatttcaataaggctttgtcttctccaatgagcttctcatataatatacgtcttagtgatggtagctctcctttccactgacatttacatctagaccccttcatttatcttcccacatctgtgttagggcgcgcgctgcgactgcgtcgctgtccgggaagggccgaagagctgctcgcccgcccggcgcccgctggggctatgggcgaggggcgcagctggacgactcagtcctgggtccccggccaggcgggcggggatggacgcggcggctcccggcactggcagccggctagtcggtcaggccgatgtgccctctgcgccgcggctgagacagcgggaaccggccccgggaggagccgcagcctgagcggccgactgaggaggcgaaggatgggcggggccacagggtcgacgac

SEQ ID NO: 16424 - RNA, 2723 nt, Homo sapiens
  source 1..2723: mol_type = other RNA
gtccacttctgcctgccctgccctaccctccccctttgggtttgtttgaggtttcattccacaaataagcagcagataaaatactttacaaggtacagcacagttgtattgaagaaaaaaaggacccaactcttactttaggagtattaggcctggacttcccctgccccatgcaataaagcaagttttatatacactccccatatttttttctaacattttcttatataaatttaaatattttacaaaaaaaggcttttttcctccaaacatataaatctgagtgaaacatagattccccacccgagaacttgtttcttcactaaaatataaatgttgtctgatattaagggtaaatgtcttttgaccactggagatcactgaagtctgaattgcaccgtggagaaggcacttgtgttttctgaggtctccagcaagtatctcagtgagcactcatagaattgctgtctgtcctccagaacccgtgccaaggcctccgagtgcccagttactgaggcagctggggaaaaacgttgagtaaacatgattctacaattacggagataaaaaataaaaacagcatggactggttctaccctagaatcaaactacaacaaaatccaaagtgttcattcatgtagattcaaaatgacttcattctgtcataaattataaaatacaaaggtggctgttttaatgacaaaactcaaaacagtactaaaaggggtttgtgtcaatggacaaaagtcagtccctctaggtagggccccaaggagcatcacccaggttgaagggtggttttcctactgctgggccagaagtgctgtcctattggccttcatcttctccagccgcttggccaggtggctgttggtcatctccatctcctcaatcttgtccagtgctgttcgtaactctcgttgtagcttccgtttttctgctttcaattcatcttcaactttctcagcattctcagcagcagttttatatctcagaacctgtccctcaagccggctaatactttgctccaaggtagttatatcctgttctgcttttgaaagcttaaatttgtattcgctaatttgtctattggcatctctctgcatttcgatgaactgcaagtctgagccattctgcagtcctgccaggtcacccactgtgccatcattcctggagcatttctgtcgttcctcctctaactgaagcttcagttttctaatctgtgacagtagttcttccttctctccagcaagttttcgtagccttacatctaatggcccttctcctgctgactccaagacctgagcagcttcctgagacacaacagtgatggctccagccactggttcatgactgacatcaccattgggagtgccatcggggattataactaagccatgtttctctcccgtcttcactgtctcctgcaggtcagccagctcctctctgagcatatctcgctcattcctaaggcaggcaatgtattctttctgtttctctagggcctcaataagctcatctctttgccgcaggccttctttaagttcttccatcttatgctgcagcacactacacatatgtttctgcctttctaactcctttgatttttcttcattttctctataaaattctgccatctgttcctcctgctcttcaataacatccttgagtgtgtctacttggtagatcaaattgttcttctcattgtctaactgtgcattggaaaccatggctttcttgtatttttcttccacttcagacaaagattcctttagttctttaagcccctgcatgtatctcccttctacatcctgtatctggtccttaaggtcatagatatcccgcaattcacttaatgaagtgtctggatctattaagctgctggtgtccccacttcctcgtctggatgagtttccacttagaggggttgttgctgaggcagaatttcgagatgaaggtcttgtataattttcagcatactgtttgtcagatttttcatccaacctgtgactgccaacacttcgaatggacaatgcatcctcaactcccagataaggacgatggtgactggaccggtgggaatacctggccctttccgaatcttccagccacttctgaatctgtccccacttccgatcaaaggaatgaagagagtactctttttgttgtcgttccagttctctcatgcgtatatctcttgcttctgcccgggcagcccgttttgctgccagccttgcctctgcctctctggcaatgttactcaaagcttcatcttctgcagaaaatcggtctttcacaggtgttcttttccttccagaagcaggagtccccatcttgtgttcttaatagtcttttaactttgaaagtgatttaactgtgttttcagcccttagtgatggtagctctcctttccactgacatttacatctagaccccttcatttatcttcccacatctgtgttagggcgcgcgctgcgactgcgtcgctgtccgggaagggccgaagagctgctcgcccgcccggcgcccgctggggctatgggcgaggggcgcagctggacgactcagtcctgggtccccggccaggcgggcggggatggacgcggcggctcccggcactggcagccggctagtcggtcaggccgatgtgccctctgcgccgcggctgagacagcgggaaccggccccgggaggagccgcagcctgagcggccgactgaggag

SEQ ID NO: 16425 - RNA, 2705 nt, Homo sapiens
  source 1..2705: mol_type = other RNA
gtccacttctgcctgccctgccctaccctccccctttgggtttgtttgaggtttcattccacaaataagcagcagataaaatactttacaaggtacagcacagttgtattgaagaaaaaaaggacccaactcttactttaggagtattaggcctggacttcccctgccccatgcaataaagcaagttttatatacactccccatatttttttctaacattttcttatataaatttaaatattttacaaaaaaaggcttttttcctccaaacatataaatctgagtgaaacatagattccccacccgagaacttgtttcttcactaaaatataaatgttgtctgatattaagggtaaatgtcttttgaccactggagatcactgaagtctgaattgcaccgtggagaaggcacttgtgttttctgaggtctccagcaagtatctcagtgagcactcatagaattgctgtctgtcctccagaacccgtgccaaggcctccgagtgcccagttactgaggcagctggggaaaaacgttgagtaaacatgattctacaattacggagataaaaaataaaaacagcatggactggttctaccctagaatcaaactacaacaaaatccaaagtgttcattcatgtagattcaaaatgacttcattctgtcataaattataaaatacaaaggtggctgttttaatgacaaaactcaaaacagtactaaaaggggtttgtgtcaatggacaaaagtcagtccctctaggtagggccccaaggagcatcacccaggttgaagggtggttttcctactgctgggccagaagtgctgtcctattggccttcatcttctccagccgcttggccaggtggctgttggtcatctccatctcctcaatcttgtccagtgctgttcgtaactctcgttgtagcttccgtttttctgctttcaattcatcttcaactttctcagcattctcagcagcagttttatatctcagaacctgtccctcaagccggctaatactttgctccaaggtagttatatcctgttctgcttttgaaagcttaaatttgtattcgctaatttgtctattggcatctctctgcatttcgatgaactgcaagtctgagccattctgcagtcctgccaggtcacccactgtgccatcattcctggagcatttctgtcgttcctcctctaactgaagcttcagttttctaatctgtgacagtagttcttccttctctccagcaagttttcgtagccttacatctaatggcccttctcctgctgactccaagacctgagcagcttcctgagacacaacagtgatggctccagccactggttcatgactgacatcaccattgggagtgccatcggggattataactaagccatgtttctctcccgtcttcactgtctcctgcaggtcagccagctcctctctgagcatatctcgctcattcctaaggcaggcaatgtattctttctgtttctctagggcctcaataagctcatctctttgccgcaggccttctttaagttcttccatcttatgctgcagcacactacacatatgtttctgcctttctaactcctttgatttttcttcattttctctataaaattctgccatctgttcctcctgctcttcaataacatccttgagtgtgtctacttggtagatcaaattgttcttctcattgtctaactgtgcattggaaaccatggctttcttgtatttttcttccacttcagacaaagattcctttagttctttaagcccctgcatgtatctcccttctacatcctgtatctggtccttaaggtcatagatatcccgcaattcacttaatgaagtgtctggatctattaagctgctggtgtccccacttcctcgtctggatgagtttccacttagaggggttgttgctgaggcagaatttcgagatgaaggtcttgtataattttcagcatactgtttgtcagatttttcatccaacctgtgactgccaacacttcgaatggacaatgcatcctcaactcccagataaggacgatggtgactggaccggtgggaatacctggccctttccgaatcttcctctttttgttgtcgttccagttctctcatgcgtatatctcttgcttctgcccgggcagcccgttttgctgccagccttgcctctgcctctctggcaatgttactcaaagcttcatcttctgcagaaaatcggtctttcacaggtgttcttttccttccagaagcaggagtccccatcttgtgttcttaatagtcttttaactttgaaagtgatttaactgtgttttcagcccttagtgatggtagctctcctttccactgacatttacatctagaccccttcatttatcttcccacatctgtgttagggcgcgcgctgcgactgcgtcgctgtccgggaagggccgaagagctgctcgcccgcccggcgcccgctggggctatgggcgaggggcgcagctggacgactcagtcctgggtccccggccaggcgggcggggatggacgcggcggctcccggcactggcagccggctagtcggtcaggccgatgtgccctctgcgccgcggctgagacagcgggaaccggccccgggaggagccgcagcctgagcggccgactgaggaggcgaaggatgggcggggccacagggtcgacgac

SEQ ID NO: 16426 - RNA, 2947 nt, Homo sapiens
  source 1..2947: mol_type = other RNA
gtccacttctgcctgccctgccctaccctccccctttgggtttgtttgaggtttcattccacaaataagcagcagataaaatactttacaaggtacagcacagttgtattgaagaaaaaaaggacccaactcttactttaggagtattaggcctggacttcccctgccccatgcaataaagcaagttttatatacactccccatatttttttctaacattttcttatataaatttaaatattttacaaaaaaaggcttttttcctccaaacatataaatctgagtgaaacatagattccccacccgagaacttgtttcttcactaaaatataaatgttgtctgatattaagggtaaatgtcttttgaccactggagatcactgaagtctgaattgcaccgtggagaaggcacttgtgttttctgaggtctccagcaagtatctcagtgagcactcatagaattgctgtctgtcctccagaacccgtgccaaggcctccgagtgcccagttactgaggcagctggggaaaaacgttgagtaaacatgattctacaattacggagataaaaaataaaaacagcatggactggttctaccctagaatcaaactacaacaaaatccaaagtgttcattcatgtagattcaaaatgacttcattctgtcataaattataaaatacaaaggtggctgttttaatgacaaaactcaaaacagtactaaaaggggtttgtgtcaatggacaaaagtcagtccctctaggtagggccccaaggagcatcacccaggttgaagggtggttttcctactgctgggccagaagtgctgtcctattggccttcatcttctccagccgcttggccaggtggctgttggtcatctccatctcctcaatcttgtccagtgctgttcgtaactctcgttgtagcttccgtttttctgctttcaattcatcttcaactttctcagcattctcagcagcagttttatatctcagaacctgtccctcaagccggctaatactttgctccaaggtagttatatcctgttctgcttttgaaagcttaaatttgtattcgctaatttgtctattggcatctctctgcatttcgatgaactgcaagtctgagccattctgcagtcctgccaggtcacccactgtgccatcattcctggagcatttctgtcgttcctcctctaactgaagcttcagttttctaatctgtgacagtagttcttccttctctccagcaagttttcgtagccttacatctaatggcccttctcctgctgactccaagacctgagcagcttcctgagacacaacagtgatggctccagccactggttcatgactgacatcaccattgggagtgccatcggggattataactaagccatgtttctctcccgtcttcactgtctcctgcaggtcagccagctcctctctgagcatatctcgctcattcctaaggcaggcaatgtattctttctgtttctctagggcctcaataagctcatctctttgccgcaggccttctttaagttcttccatcttatgctgcagcacactacacatatgtttctgcctttctaactcctttgatttttcttcattttctctataaaattctgccatctgttcctcctgctcttcaataacatccttgagtgtgtctacttggtagatcaaattgttcttctcattgtctaactgtgcattggaaaccatggctttcttgtatttttcttccacttcagacaaagattcctttagttctttaagcccctgcatgtatctcccttctacatcctgtatctggtccttaaggtcatagatatcccgcaattcacttaatgaagtgtctggatctattaagctgctggtgtccccacttcctcgtctggatgagtttccacttagaggggttgttgctgaggcagaatttcgagatgaaggtcttgtataattttcagcatactgtttgtcagatttttcatccaacctgtgactgccaacacttcgaatggacaatgcatcctcaactcccagataaggacgatggtgactggaccggtgggaatacctggccctttccgaatcttcctctttttgttgtcgttccagttctctcatgcgtatatctcttgcttctgcccgggcagcccgttttgctgccagccttgcctctgcctctctggcaatgttactcaaagcttcatcttctgcagaaaatcggtctttcacaggtgttcttttccttccagaagcaggagtccccatcttgtgttcttaatagtcttttaactttgaaagtgatttaactgtgttttcagcccttagtgatggtagctctcctttccactgacatttacatctagaccccttcatttatcttcccacatcttttccccagcgcggtggaagggtgagcgttagaaatcagacgggatgtctgagaacgccgcaggcagggggcgaccccagcccgggagcccgccgcgggccggccagtccccagggaagcccggccccctagccgaggtcggaggcggcgcggatcccacgggactgcggaggccgggaaaaaggttcccaactccccgctccctgctcccaccgggctggcgggaggagcggcccttacctgtgttagggcgcgcgctgcgactgcgtcgctgtccgggaagggccgaagagctgctcgcccgcccggcgcccgctggggctatgggcgaggggcgcagctggacgactcagtcctgggtccccggccaggcgggcggggatggacgcggcggctcccggcactggcagccggctagtcggtcaggccgatgtgccctctgcgccgcggctgagacagcgggaaccggccccgggaggagccgcagcctgagcggccgactgaggaggcgaaggatgggcggggccacagggtcgacgac

SEQ ID NO: 16427 - RNA, 2476 nt, Homo sapiens
  source 1..2476: mol_type = other RNA
gtccacttctgcctgccctgccctaccctccccctttgggtttgtttgaggtttcattccacaaataagcagcagataaaatactttacaaggtacagcacagttgtattgaagaaaaaaaggacccaactcttactttaggagtattaggcctggacttcccctgccccatgcaataaagcaagttttatatacactccccatatttttttctaacattttcttatataaatttaaatattttacaaaaaaaggcttttttcctccaaacatataaatctgagtgaaacatagattccccacccgagaacttgtttcttcactaaaatataaatgttgtctgatattaagggtaaatgtcttttgaccactggagatcactgaagtctgaattgcaccgtggagaaggcacttgtgttttctgaggtctccagcaagtatctcagtgagcactcatagaattgctgtctgtcctccagaacccgtgccaaggcctccgagtgcccagttactgaggcagctggggaaaaacgttgagtaaacatgattctacaattacggagataaaaaataaaaacagcatggactggttctaccctagaatcaaactacaacaaaatccaaagtgttcattcatgtagattcaaaatgacttcattctgtcataaattataaaatacaaaggtggctgttttaatgacaaaactcaaaacagtactaaaaggggtttgtgtcaatggacaaaagtcagtccctctaggtagggccccaaggagcatcacccaggttgaagggtggttttcctactgctgggccagaagtgctgtcctattggccttcatcttctccagccgcttggccaggtggctgttggtcatctccatctcctcaatcttgtccagtgctgttcgtaactctcgttgtagcttccgtttttctgctttcaattcatcttcaactttctcagcattctcagcagcagttttatatctcagaacctgtccctcaagccggctaatactttgctccaaggtagttatatcctgttctgcttttgaaagcttaaatttgtattcgctaatttgtctattggcatctctctgcatttcgatgaactgcaagtctgagccattctgcagtcctgccaggtcacccactgtgccatcattcctggagcatttctgtcgttcctcctctaactgaagcttcagttttctaatctgtgacagtagttcttccttctctccagcaagttttcgtagccttacatctaatggcccttctcctgctgactccaagacctgagcagcttcctgagacacaacagtgatggctccagccactggttcatgactgacatcaccattgggagtgccatcggggattataactaagccatgtttctctcccgtcttcactgtctcctgcaggtcagccagctcctctctgagcatatctcgctcattcctaaggcaggcaatgtattctttctgtttctctagggcctcaataagctcatctctttgccgcaggccttctttaagttcttccatcttatgctgcagcacactacacatatgtttctgcctttctaactcctttgatttttcttcattttctctataaaattctgccatctgttcctcctgctcttcaataacatccttgagtgtgtctacttggtagatcaaattgttcttctcattgtctaactgtgcattggaaaccatggctttcttgtatttttcttccacttcagacaaagattcctttagttctttaagcccctgcatgtatctcccttctacatcctgtatctggtccttaaggtcatagatatcccgcaattcacttaatgaagtgtctggatctattaagctgctggtgtccccacttcctcgtctggatgagtttccacttagaggggttgttgctgaggcagaatttcgagatgaaggtcttgtataattttcagcatactgtttgtcagatttttcatccaactctttttgttgtcgttccagttctctcatgcgtatatctcttgcttctgcccgggcagcccgttttgctgccagccttgcctctgcctctctggcaatgttactcaaagcttcatcttctgcagaaaatcggtctttcacaggtgttcttttccttccagaagcaggagtccccatcttgtgttcttaatagtcttttaactttgaaagtgatttaactgtgttttcagcccttagtgatggtagctctcctttccactgacatttacatctagaccccttcatttatcttcccacatcattcttcacgatgataaatatccagcaacagacctaacaaaacataatacaacacttcctataaaatgagtaaagaatgccatctcattaggcagatacgaacttaggtttcctctatttcaattttcagattcatagcaatgattcacaaagtgagtgatctaccttcgaaa

SEQ ID NO: 16428 - RNA, 2603 nt, Homo sapiens
  source 1..2603: mol_type = other RNA
gtccacttctgcctgccctgccctaccctccccctttgggtttgtttgaggtttcattccacaaataagcagcagataaaatactttacaaggtacagcacagttgtattgaagaaaaaaaggacccaactcttactttaggagtattaggcctggacttcccctgccccatgcaataaagcaagttttatatacactccccatatttttttctaacattttcttatataaatttaaatattttacaaaaaaaggcttttttcctccaaacatataaatctgagtgaaacatagattccccacccgagaacttgtttcttcactaaaatataaatgttgtctgatattaagggtaaatgtcttttgaccactggagatcactgaagtctgaattgcaccgtggagaaggcacttgtgttttctgaggtctccagcaagtatctcagtgagcactcatagaattgctgtctgtcctccagaacccgtgccaaggcctccgagtgcccagttactgaggcagctggggaaaaacgttgagtaaacatgattctacaattacggagataaaaaataaaaacagcatggactggttctaccctagaatcaaactacaacaaaatccaaagtgttcattcatgtagattcaaaatgacttcattctgtcataaattataaaatacaaaggtggctgttttaatgacaaaactcaaaacagtactaaaaggggtttgtgtcaatggacaaaagtcagtccctctaggtagggccccaaggagcatcacccaggttgaagggtggttttcctactgctgggccagaagtgctgtcctattggccttcatcttctccagccgcttggccaggtggctgttggtcatctccatctcctcaatcttgtccagtgctgttcgtaactctcgttgtagcttccgtttttctgctttcaattcatcttcaactttctcagcattctcagcagcagttttatatctcagaacctgtccctcaagccggctaatactttgctccaaggtagttatatcctgttctgcttttgaaagcttaaatttgtattcgctaatttgtctattggcatctctctgcatttcgatgaactgcaagtctgagccattctgcagtcctgccaggtcacccactgtgccatcattcctggagcatttctgtcgttcctcctctaactgaagcttcagttttctaatctgtgacagtagttcttccttctctccagcaagttttcgtagccttacatctaatggcccttctcctgctgactccaagacctgagcagcttcctgagacacaacagtgatggctccagccactggttcatgactgacatcaccattgggagtgccatcggggattataactaagccatgtttctctcccgtcttcactgtctcctgcaggtcagccagctcctctctgagcatatctcgctcattcctaaggcaggcaatgtattctttctgtttctctagggcctcaataagctcatctctttgccgcaggccttctttaagttcttccatcttatgctgcagcacactacacatatgtttctgcctttctaactcctttgatttttcttcattttctctataaaattctgccatctgttcctcctgctcttcaataacatccttgagtgtgtctacttggtagatcaaattgttcttctcattgtctaactgtgcattggaaaccatggctttcttgtatttttcttccacttcagacaaagattcctttagttctttaagcccctgcatgtatctcccttctacatcctgtatctggtccttaaggtcatagatatcccgcaattcacttaatgaagtgtctggatctattaagctgctggtgtccccacttcctcgtctggatgagtttccacttagaggggttgttgctgaggcagaatttcgagatgaaggtcttgtataattttcagcatactgtttgtcagatttttcatccaactctttttgttgtcgttccagttctctcatgcgtatatctcttgcttctgcccgggcagcccgttttgctgccagccttgcctctgcctctctggcaatgttactcaaagcttcatcttctgcagaaaatcggtctttcacaggtgttcttttccttccagaagcaggagtccccatcttgtgttcttaatagtcttttaactttgaaagtgatttaactgtgttttcagcccttagtgatggtagctctcctttccactgacatttacatctagaccccttcatttatcttcccacatctgtgttagggcgcgcgctgcgactgcgtcgctgtccgggaagggccgaagagctgctcgcccgcccggcgcccgctggggctatgggcgaggggcgcagctggacgactcagtcctgggtccccggccaggcgggcggggatggacgcggcggctcccggcactggcagccggctagtcggtcaggccgatgtgccctctgcgccgcggctgagacagcgggaaccggccccgggaggagccgcagcctgagcggccgactgaggaggcgaaggatgggcggggccacagggtcgacgac

SEQ ID NO: 16429 - RNA, 2845 nt, Homo sapiens
  source 1..2845: mol_type = other RNA
gtccacttctgcctgccctgccctaccctccccctttgggtttgtttgaggtttcattccacaaataagcagcagataaaatactttacaaggtacagcacagttgtattgaagaaaaaaaggacccaactcttactttaggagtattaggcctggacttcccctgccccatgcaataaagcaagttttatatacactccccatatttttttctaacattttcttatataaatttaaatattttacaaaaaaaggcttttttcctccaaacatataaatctgagtgaaacatagattccccacccgagaacttgtttcttcactaaaatataaatgttgtctgatattaagggtaaatgtcttttgaccactggagatcactgaagtctgaattgcaccgtggagaaggcacttgtgttttctgaggtctccagcaagtatctcagtgagcactcatagaattgctgtctgtcctccagaacccgtgccaaggcctccgagtgcccagttactgaggcagctggggaaaaacgttgagtaaacatgattctacaattacggagataaaaaataaaaacagcatggactggttctaccctagaatcaaactacaacaaaatccaaagtgttcattcatgtagattcaaaatgacttcattctgtcataaattataaaatacaaaggtggctgttttaatgacaaaactcaaaacagtactaaaaggggtttgtgtcaatggacaaaagtcagtccctctaggtagggccccaaggagcatcacccaggttgaagggtggttttcctactgctgggccagaagtgctgtcctattggccttcatcttctccagccgcttggccaggtggctgttggtcatctccatctcctcaatcttgtccagtgctgttcgtaactctcgttgtagcttccgtttttctgctttcaattcatcttcaactttctcagcattctcagcagcagttttatatctcagaacctgtccctcaagccggctaatactttgctccaaggtagttatatcctgttctgcttttgaaagcttaaatttgtattcgctaatttgtctattggcatctctctgcatttcgatgaactgcaagtctgagccattctgcagtcctgccaggtcacccactgtgccatcattcctggagcatttctgtcgttcctcctctaactgaagcttcagttttctaatctgtgacagtagttcttccttctctccagcaagttttcgtagccttacatctaatggcccttctcctgctgactccaagacctgagcagcttcctgagacacaacagtgatggctccagccactggttcatgactgacatcaccattgggagtgccatcggggattataactaagccatgtttctctcccgtcttcactgtctcctgcaggtcagccagctcctctctgagcatatctcgctcattcctaaggcaggcaatgtattctttctgtttctctagggcctcaataagctcatctctttgccgcaggccttctttaagttcttccatcttatgctgcagcacactacacatatgtttctgcctttctaactcctttgatttttcttcattttctctataaaattctgccatctgttcctcctgctcttcaataacatccttgagtgtgtctacttggtagatcaaattgttcttctcattgtctaactgtgcattggaaaccatggctttcttgtatttttcttccacttcagacaaagattcctttagttctttaagcccctgcatgtatctcccttctacatcctgtatctggtccttaaggtcatagatatcccgcaattcacttaatgaagtgtctggatctattaagctgctggtgtccccacttcctcgtctggatgagtttccacttagaggggttgttgctgaggcagaatttcgagatgaaggtcttgtataattttcagcatactgtttgtcagatttttcatccaactctttttgttgtcgttccagttctctcatgcgtatatctcttgcttctgcccgggcagcccgttttgctgccagccttgcctctgcctctctggcaatgttactcaaagcttcatcttctgcagaaaatcggtctttcacaggtgttcttttccttccagaagcaggagtccccatcttgtgttcttaatagtcttttaactttgaaagtgatttaactgtgttttcagcccttagtgatggtagctctcctttccactgacatttacatctagaccccttcatttatcttcccacatcttttccccagcgcggtggaagggtgagcgttagaaatcagacgggatgtctgagaacgccgcaggcagggggcgaccccagcccgggagcccgccgcgggccggccagtccccagggaagcccggccccctagccgaggtcggaggcggcgcggatcccacgggactgcggaggccgggaaaaaggttcccaactccccgctccctgctcccaccgggctggcgggaggagcggcccttacctgtgttagggcgcgcgctgcgactgcgtcgctgtccgggaagggccgaagagctgctcgcccgcccggcgcccgctggggctatgggcgaggggcgcagctggacgactcagtcctgggtccccggccaggcgggcggggatggacgcggcggctcccggcactggcagccggctagtcggtcaggccgatgtgccctctgcgccgcggctgagacagcgggaaccggccccgggaggagccgcagcctgagcggccgactgaggaggcgaaggatgggcggggccacagggtcgacgac

SEQ ID NO: 16430 - RNA, 3266 nt, Homo sapiens
  source 1..3266: mol_type = other RNA
gtccacttctgcctgccctgccctaccctccccctttgggtttgtttgaggtttcattccacaaataagcagcagataaaatactttacaaggtacagcacagttgtattgaagaaaaaaaggacccaactcttactttaggagtattaggcctggacttcccctgccccatgcaataaagcaagttttatatacactccccatatttttttctaacattttcttatataaatttaaatattttacaaaaaaaggcttttttcctccaaacatataaatctgagtgaaacatagattccccacccgagaacttgtttcttcactaaaatataaatgttgtctgatattaagggtaaatgtcttttgaccactggagatcactgaagtctgaattgcaccgtggagaaggcacttgtgttttctgaggtctccagcaagtatctcagtgagcactcatagaattgctgtctgtcctccagaacccgtgccaaggcctccgagtgcccagttactgaggcagctggggaaaaacgttgagtaaacatgattctacaattacggagataaaaaataaaaacagcatggactggttctaccctagaatcaaactacaacaaaatccaaagtgttcattcatgtagattcaaaatgacttcattctgtcataaattataaaatacaaaggtggctgttttaatgacaaaactcaaaacagtactaaaaggggtttgtgtcaatggacaaaagtcagtccctctaggtagggccccaaggagcatcacccaggttgaagggtggttttcctactgctgggccagaagtgctgtcctattggccttcatcttctccagccgcttggccaggtggctgttggtcatctccatctcctcaatcttgtccagtgctgttcgtaactctcgttgtagcttccgtttttctgctttcaattcatcttcaactttctcagcattctcagcagcagttttatatctcagaacctgtccctcaagccggctaatactttgctccaaggtagttatatcctgttctgcttttgaaagcttaaatttgtattcgctaatttgtctattggcatctctctgcatttcgatgaactgcaagtctgagccattctgcagtcctgccaggtcacccactgtgccatcattcctggagcatttctgtcgttcctcctctaactgaagcttcagttttctaatctgtgacagtagttcttccttctctccagcaagttttcgtagccttacatctaatggcccttctcctgctgactccaagacctgagcagcttcctgagacacaacagtgatggctccagccactggttcatgactgacatcaccattgggagtgccatcggggattataactaagccatgtttctctcccgtcttcactgtctcctgcaggtcagccagctcctctctgagcatatctcgctcattcctaaggcaggcaatgtattctttctgtttctctagggcctcaataagctcatctctttgccgcaggccttctttaagttcttccatcttatgctgcagcacactacacatatgtttctgcctttctaactcctttgatttttcttcattttctctataaaattctgccatctgttcctcctgctcttcaataacatccttgagtgtgtctacttggtagatcaaattgttcttctcattgtctaactgtgcattggaaaccatggctttcttgtatttttcttccacttcagacaaagattcctttagttctttaagcccctgcatgtatctcccttctacatcctgtatctggtccttaaggtcatagatatcccgcaattcacttaatgaagtgtctggatctattaagctgctggtgtccccacttcctcgtctggatgagtttccacttagaggggttgttgctgaggcagaatttcgagatgaaggtcttgtataattttcagcatactgtttgtcagatttttcatccaagctggacaaatctgggatactgatatcatccacctcagagacaacacttcccctacgattggagcgactgaaataatcagcggcagataccacactctcccttcgtccacgactggcacgatcagaagacacaatgcttgcagtgtcatcgttggtaaaccctggactgcttcgggctgaacttattcttgatgaataataactgcattcagatggagttcgaggaccataagggttatataatccaccattgtacaatgatgccagactggcacttctcagcagaccagaatttgcagtaggagaggccctgtcactcttatatgttgccagagggtcactgtacagggaagaagactgccgagtgtagtaggcagaggtgggtttgctatgtctaagactgctatagtttctctggtcaaagtagaggccactcagtaggtctttatgagaatcagaagacctcttcttcattccatgagagtgactgtaagaatgatttaatgatgaaagtcttgatgatctatccttgaacatatcatacctgtgactgccaacacttcgaatggacaatgcatcctcaactcccagataaggacgatggtgactggaccggtgggaatacctggccctttccgaatcttccagccacttctgaatctgtccccacttccgatcaaaggaatgaagagagtactctttttgttgtcgttccagttctctcatgcgtatatctcttgcttctgcccgggcagcccgttttgctgccagccttgcctctgcctctctggcaatgttactcaaagcttcatcttctgcagaaaatcggtctttcacaggtgttcttttccttccagaagcaggagtccccatcttgtgttcttaatagtcttttaactttgaaagtgatttaactgtgttttcagcccttagtgatggtagctctcctttccactgacatttacatctagaccccttcatttatcttcccacatctgtgttagggcgcgcgctgcgactgcgtcgctgtccgggaagggccgaagagctgctcgcccgcccggcgcccgctggggctatgggcgaggggcgcagctggacgactcagtcctgggtccccggccaggcgggcggggatggacgcggcggctcccggcactggcagccggctagtcggtcaggccgatgtgccctctgcgccgcggctgagacagcgggaaccggccccgggaggagccgcagcctgagcggccgactgaggag

SEQ ID NO: 16431 - RNA, 3031 nt, Homo sapiens
  source 1..3031: mol_type = other RNA
gtccacttctgcctgccctgccctaccctccccctttgggtttgtttgaggtttcattccacaaataagcagcagataaaatactttacaaggtacagcacagttgtattgaagaaaaaaaggacccaactcttactttaggagtattaggcctggacttcccctgccccatgcaataaagcaagttttatatacactccccatatttttttctaacattttcttatataaatttaaatattttacaaaaaaaggcttttttcctccaaacatataaatctgagtgaaacatagattccccacccgagaacttgtttcttcactaaaatataaatgttgtctgatattaagggtaaatgtcttttgaccactggagatcactgaagtctgaattgcaccgtggagaaggcacttgtgttttctgaggtctccagcaagtatctcagtgagcactcatagaattgctgtctgtcctccagaacccgtgccaaggcctccgagtgcccagttactgaggcagctggggaaaaacgttgagtaaacatgattctacaattacggagataaaaaataaaaacagcatggactggttctaccctagaatcaaactacaacaaaatccaaagtgttcattcatgtagattcaaaatgacttcattctgtcataaattataaaatacaaaggtggctgttttaatgacaaaactcaaaacagtactaaaaggggtttgtgtcaatggacaaaagtcagtccctctaggtagggccccaaggagcatcacccaggttgaagggtggttttcctactgctgggccagaagtgctgtcctattggccttcatcttctccagccgcttggccaggtggctgttggtcatctccatctcctcaatcttgtccagtgctgttcgtaactctcgttgtagcttccgtttttctgctttcaattcatcttcaactttctcagcattctcagcagcagttttatatctcagaacctgtccctcaagccggctaatactttgctccaaggtagttatatcctgttctgcttttgaaagcttaaatttgtattcgctaatttgtctattggcatctctctgcatttcgatgaactgcaagtctgagccattctgcagtcctgccaggtcacccactgtgccatcattcctggagcatttctgtcgttcctcctctaactgaagcttcagttttctaatctgtgacagtagttcttccttctctccagcaagttttcgtagccttacatctcaataagctcatctctttgccgcaggccttctttaagttcttccatcttatgctgcagcacactacacatatgtttctgcctttctaactcctttgatttttcttcattttctctataaaattctgccatctgttcctcctgctcttcaataacatccttgagtgtgtctacttggtagatcaaattgttcttctcattgtctaactgtgcattggaaaccatggctttcttgtatttttcttccacttcagacaaagattcctttagttctttaagcccctgcatgtatctcccttctacatcctgtatctggtccttaaggtcatagatatcccgcaattcacttaatgaagtgtctggatctattaagctgctggtgtccccacttcctcgtctggatgagtttccacttagaggggttgttgctgaggcagaatttcgagatgaaggtcttgtataattttcagcatactgtttgtcagatttttcatccaagctggacaaatctgggatactgatatcatccacctcagagacaacacttcccctacgattggagcgactgaaataatcagcggcagataccacactctcccttcgtccacgactggcacgatcagaagacacaatgcttgcagtgtcatcgttggtaaaccctggactgcttcgggctgaacttattcttgatgaataataactgcattcagatggagttcgaggaccataagggttatataatccaccattgtacaatgatgccagactggcacttctcagcagaccagaatttgcagtaggagaggccctgtcactcttatatgttgccagagggtcactgtacagggaagaagactgccgagtgtagtaggcagaggtgggtttgctatgtctaagactgctatagtttctctggtcaaagtagaggccactcagtaggtctttatgagaatcagaagacctcttcttcattccatgagagtgactgtaagaatgatttaatgatgaaagtcttgatgatctatccttgaacatatcatacctgtgactgccaacacttcgaatggacaatgcatcctcaactcccagataaggacgatggtgactggaccggtgggaatacctggccctttccgaatcttccagccacttctgaatctgtccccacttccgatcaaaggaatgaagagagtactctttttgttgtcgttccagttctctcatgcgtatatctcttgcttctgcccgggcagcccgttttgctgccagccttgcctctgcctctctggcaatgttactcaaagcttcatcttctgcagaaaatcggtctttcacaggtgttcttttccttccagaagcaggagtccccatcttgtgttcttaatagtcttttaactttgaaagtgatttaactgtgttttcagcccttagtgatggtagctctcctttccactgacatttacatctagaccccttcatttatcttcccacatctgtgttagggcgcgcgctgcgactgcgtcgctgtccgggaagggccgaagagctgctcgcccgcccggcgcccgctggggctatgggcgaggggcgcagctggacgactcagtcctgggtccccggccaggcgggcggggatggacgcggcggctcccggcactggcagccggctagtcggtcaggccgatgtgccctctgcgccgcggctgagacagcgggaaccggccccgggaggagccgcagcctgagcggccgactgaggag

SEQ ID NO: 16432 - RNA, 4576 nt, Homo sapiens
  source 1..4576: mol_type = other RNA
gtccacttctgcctgccctgccctccatatccccctgccaccatccacacaccaatgggaatgccgctctggcccacagaggctcctctccctcccggcatccatgtgacgtgtgtcataccgcaccgtggcaggctggggaaggggcacagggtcaccctgaaactgtggaatgcacctcctccccctgcaatcccctccccaacccagaggggaaaatgaaggtcaccctgatttgactctccatgtaaaatggcattttcttccataacatcccatatcaatgtgtcaattttctattaattttactggggaagtgtcttccccttgtttctcactctgcctcctcctctgtgttattatgggcttgaggggcaggggtagctattgctcatgacttttactacaagataaccagacttcctaagccctccatattgggaccaatttctgctgaatgccaggtgatgagaggtttcagcccctggcgtgggtggatgacgtcagaccagggcagcagaggactctcattccacaagctccctcaggactgagcacttgctccgggtctcctgaagccccatgtccatctccttgtctgccctgccagtctagcagacttgggctgagaaccagacctttgcccttggcccagcctcgccttccccactgggtctctagatttctagattccccatagggtatgccagcaaggagaggatatgagggcccaagaaaactcaggaaagtttctatcaccaagggcagaacacgaacatcttgaggctaaaggagctgcatggttgctaccaacaaaggagaccgacggtgtgcagttgattcccatgtttttactgcacttcacccccaaattcccagcaaggtctaaggcttcgccaggaacccttgtcttcttgccaaaggcatgtcagggccatcctgcaatactcatgaggttgcctgtcccttcatgcccctcaccccaccccaggattaatcatcaaagaaggactgtctacatgtcctcctccctgtgcttaggaagagagacaaataagagaatgagaaggctgggaaggcccttagcggtcacatcaagcaactgtccttgccaaggttttatggaggaggaaactgaggccgccttgtgctgagtggcttacccgtgagcagccggcactccatagggccacagcagagactgtttcttcgtggcacggaaggacatctctgcttgctggtcccacgggctaggacagcccctattgacgttgcactatagctgcatgtgacctttaaccaatggtaaaatagccggatttgtttccacctccttctgaggttctgacctggagatgccattgcttcttatctgcctcctttcaaggcccagctcagatcccatggccctggagagacggttctgggctcctcagttggtggagtctctcctccctcctcaagggccagagtccttggttagtcgccaagaagtgaagccagcaagcccagagccctggggaaagcgccttgccttggaggaggaaagaggtggagaagctgcccctggacagagggtcgccagccgaatccttccagggggtacctggtttgaggggatgatcaaagtgtattgtgacctcaggagtgcaaggatgggcctctgtcctctccaagggctagagctcagccaggaaagccaaggcccccacatccgcacacctccagctctcgtggcctgctgaggtgtctgctgcagccccagccaggaccctctgctgttgctgcaattttgagggctctcggactcctcttgctcatgaagaattgtggttctgtgagcaacctctctgcagaaggggctgtcagtaccatcctgatctgactgggaaagcctcctcccgaggcaggccaggcagctgtcacctctcccacctcttctcaacagagttccttcaatttcctttggtgctgccaccatcaaccctgttacttcctgggctctttccagtgtcataagcagacgaatgtaccaagctggaaaagcaaggagcgtttgtcttagaaaggacggaaccgcaacataatggaggagagaagcccaggagtaatactgggtggccatgccgggtgcctgggctggtcctcagaaccaggagcctcacacatctagtccggtgcccagaggtgccccagccagtactaaactgacacagacggaggcagcagtctatgtagtttcaggagggtctgaagtaagccctcttagcaaaattgttgaagggacagtggctggaaattaaccaccttacatctccctttgtcatgacactcaaaccaccttgctgcttgcttcttcagtgaatagaatgaccatattttcttgttctatccaggacactttgcaattaagaagggccctggtagtcagtaggctgtgacagcagatgtcaacctggcaaaccagcaggtggtcacagtgacaatgacccaatacccacgtcatcctccagcccttccaagccaagctctggcaacagctcaacccctcctggtgccttgtagctgcagccattcaccaatggcctcaggtgtccacagggccaggtggacattgtgtggagaacaaagtgaacacgcccctgttctcacctccatgcacctgggcgagtgggatatgatcagaacacaaatgacaactctcaccgaaggcaggacagacaggccagcggaaggcagaaatgaagggcaggggacattcaaaggatagaaagatcttgaataaacaaacatttggagggaatttttccccgacactattttaagatggagaggctgggtcgccagggttaccaggccattctggtgatttgactttaaatgctgggattctgactttaaattcataacaacatctttcctcggccctggtgggttaaagaaaatgctttagagcaaatttagtgttttctcccattcacagtatctggcccacaaggcttgtgggttaaagcacactcctgatcttcatttgataacctcatctctctcctctcttttggtgcttattgtaaagtaggaacagcagcctcattacatggggaggagcagtatgtccagggctgcaaacaaattgcgcaggtccattgcggccccgttggggtcaagggcacatgtgcatgactggatgcagcaaaagtcacagctaatgcaccccgatggtgatccagatgtgatgtgaggctcagtgggtacttagagatttttcacagccaagttaaccagtcacccaaccctcctgcccttcccagggcatggcagaaataaaaggcatccctatttaaaatgacacacgtgtgagtgggtttgaggattccagatgactcacaggatcctgtacatttgtatatagtcaaatggtcttcatctcctgccagcaaaccaccccgctctaaacctacaacagtcgaggaagacaaacccatcacgaccaccttctaagaagacacagccaagtcccagggctcactgtaagatcacaaatgcagtgaaactgcttgctaagagacatttttcttgcactccactcattccaaagacaaagcaatttattgcaaagtctgccaaaataaacgtgcctgcagctcccccagccagtgggaaagcacttgggctgggatgggagtaaggagatcgggtgcttgctccggccacagcgtgctagcagagtgaccgtaggcaagtgccgcccatgctctgagcctccagtccctcatgtgtgacctggggcaggcactgcctacctcccaggtgatatgagggctatctctgtggaagcacttggaacacagtaaagagccatgcaaaggctagacaatgcgattgctagtgtttgctgttcagaaaaacaaaaaacaaaaaataaccttgcttttcatagacaaacctcaattacatggaatcacttaagaatggttcgttaaaatttctggtgaaattaggttcaaagaggacctccttggaggcatgaagaaggcctgactgataaacactgtggacactgagtaatgaagatgtggaaatggtggccagcttggggaaagacatgaggatagatctaggaagttgctttttcaaactaaagtccataaatgttcataagagatttttttccctttctcctagaaaagtcagcaacttaaattatttttgctttaaaattccagttccccatattgctcgttaaatgaggtttttctcttcagagggctccagcctgcaatgtttcctccatcctggtcctgcccccacctccctccttctatctcctgcccccctgtgcccttggagacacgctgggcagactccccatgtgatcaatctgacgtcttaagtttaaacgtcattacctcagtatatcagcagaaaaagttctatttcattgtgtcttgtggcaaacttcagttcggttaatggagggtttcgtatacttttaaaagtaagtcaggctgggtgcagtggctcacccctgtaatccccagcactttgggaggccaagatgggaggatcacttcag

SEQ ID NO: 16433 - RNA, 4582 nt, Homo sapiens
  source 1..4582: mol_type = other RNA
gtccacttctgcctgccctgccctccatatccccctgccaccatccacacaccaatgggaatgccgctctggcccacagaggctcctctccctcccggcatccatgtgacgtgtgtcataccgcaccgtggcaggctggggaaggggcacagggtcaccctgaaactgtggaatgcacctcctccccctgcaatcccctccccaacccagaggggaaaatgaaggtcaccctgatttgactctccatgtaaaatggcattttcttccataacatcccatatcaatgtgtcaattttctattaattttactggggaagtgtcttccccttgtttctcactctgcctcctcctctgtgttattatgggcttgaggggcaggggtagctattgctcatgacttttactacaagataaccagacttcctaagccctccatattgggaccaatttctgctgaatgccaggtgatgagaggtttcagcccctggcgtgggtggatgacgtcagaccagggcagcagaggactctcattccacaagctccctcaggactgagcacttgctccgggtctcctgaagccccatgtccatctccttgtctgccctgccagtctagcagacttgggctgagaaccagacctttgcccttggcccagcctcgccttccccactgggtctctagatttctagattccccatagggtatgccagcaaggagaggatatgagggcccaagaaaactcaggaaagtttctatcaccaagggcagaacacgaacatcttgaggctaaaggagctgcatggttgctaccaacaaaggagaccgacggtgtgcagttgattcccatgtttttactgcacttcacccccaaattcccagcaaggtctaaggcttcgccaggaacccttgtcttcttgccaaaggcatgtcagggccatcctgcaatactcatgaggttgcctgtcccttcatgcccctcaccccaccccaggattaatcatcaaagaaggactgtctacatgtcctcctccctgtgcttaggaagagagacaaataagagaatgagaaggctgggaaggcccttagcggtcacatcaagcaactgtccttgccaaggttttatggaggaggaaactgaggccgccttgtgctgagtggcttacccgtgagcagccggcactccatagggccacagcagagactgtttcttcgtggcacggaaggacatctctgcttgctggtcccacgggctaggacagcccctattgacgttgcactatagctgcatgtgacctttaaccaatggtaaaatagccggatttgtttccacctccttctgaggttctgacctggagatgccattgcttcttatctgcctcctttcaaggcccagctcagatcccatggccctggagagacggttctgggctcctcagttggtggagtctctcctccctgcaactcctcaagggccagagtccttggttagtcgccaagaagtgaagccagcaagcccagagccctggggaaagcgccttgccttggaggaggaaagaggtggagaagctgcccctggacagagggtcgccagccgaatccttccagggggtacctggtttgaggggatgatcaaagtgtattgtgacctcaggagtgcaaggatgggcctctgtcctctccaagggctagagctcagccaggaaagccaaggcccccacatccgcacacctccagctctcgtggcctgctgaggtgtctgctgcagccccagccaggaccctctgctgttgctgcaattttgagggctctcggactcctcttgctcatgaagaattgtggttctgtgagcaacctctctgcagaaggggctgtcagtaccatcctgatctgactgggaaagcctcctcccgaggcaggccaggcagctgtcacctctcccacctcttctcaacagagttccttcaatttcctttggtgctgccaccatcaaccctgttacttcctgggctctttccagtgtcataagcagacgaatgtaccaagctggaaaagcaaggagcgtttgtcttagaaaggacggaaccgcaacataatggaggagagaagcccaggagtaatactgggtggccatgccgggtgcctgggctggtcctcagaaccaggagcctcacacatctagtccggtgcccagaggtgccccagccagtactaaactgacacagacggaggcagcagtctatgtagtttcaggagggtctgaagtaagccctcttagcaaaattgttgaagggacagtggctggaaattaaccaccttacatctccctttgtcatgacactcaaaccaccttgctgcttgcttcttcagtgaatagaatgaccatattttcttgttctatccaggacactttgcaattaagaagggccctggtagtcagtaggctgtgacagcagatgtcaacctggcaaaccagcaggtggtcacagtgacaatgacccaatacccacgtcatcctccagcccttccaagccaagctctggcaacagctcaacccctcctggtgccttgtagctgcagccattcaccaatggcctcaggtgtccacagggccaggtggacattgtgtggagaacaaagtgaacacgcccctgttctcacctccatgcacctgggcgagtgggatatgatcagaacacaaatgacaactctcaccgaaggcaggacagacaggccagcggaaggcagaaatgaagggcaggggacattcaaaggatagaaagatcttgaataaacaaacatttggagggaatttttccccgacactattttaagatggagaggctgggtcgccagggttaccaggccattctggtgatttgactttaaatgctgggattctgactttaaattcataacaacatctttcctcggccctggtgggttaaagaaaatgctttagagcaaatttagtgttttctcccattcacagtatctggcccacaaggcttgtgggttaaagcacactcctgatcttcatttgataacctcatctctctcctctcttttggtgcttattgtaaagtaggaacagcagcctcattacatggggaggagcagtatgtccagggctgcaaacaaattgcgcaggtccattgcggccccgttggggtcaagggcacatgtgcatgactggatgcagcaaaagtcacagctaatgcaccccgatggtgatccagatgtgatgtgaggctcagtgggtacttagagatttttcacagccaagttaaccagtcacccaaccctcctgcccttcccagggcatggcagaaataaaaggcatccctatttaaaatgacacacgtgtgagtgggtttgaggattccagatgactcacaggatcctgtacatttgtatatagtcaaatggtcttcatctcctgccagcaaaccaccccgctctaaacctacaacagtcgaggaagacaaacccatcacgaccaccttctaagaagacacagccaagtcccagggctcactgtaagatcacaaatgcagtgaaactgcttgctaagagacatttttcttgcactccactcattccaaagacaaagcaatttattgcaaagtctgccaaaataaacgtgcctgcagctcccccagccagtgggaaagcacttgggctgggatgggagtaaggagatcgggtgcttgctccggccacagcgtgctagcagagtgaccgtaggcaagtgccgcccatgctctgagcctccagtccctcatgtgtgacctggggcaggcactgcctacctcccaggtgatatgagggctatctctgtggaagcacttggaacacagtaaagagccatgcaaaggctagacaatgcgattgctagtgtttgctgttcagaaaaacaaaaaacaaaaaataaccttgcttttcatagacaaacctcaattacatggaatcacttaagaatggttcgttaaaatttctggtgaaattaggttcaaagaggacctccttggaggcatgaagaaggcctgactgataaacactgtggacactgagtaatgaagatgtggaaatggtggccagcttggggaaagacatgaggatagatctaggaagttgctttttcaaactaaagtccataaatgttcataagagatttttttccctttctcctagaaaagtcagcaacttaaattatttttgctttaaaattccagttccccatattgctcgttaaatgaggtttttctcttcagagggctccagcctgcaatgtttcctccatcctggtcctgcccccacctccctccttctatctcctgcccccctgtgcccttggagacacgctgggcagactccccatgtgatcaatctgacgtcttaagtttaaacgtcattacctcagtatatcagcagaaaaagttctatttcattgtgtcttgtggcaaacttcagttcggttaatggagggtttcgtatacttttaaaagtaagtcaggctgggtgcagtggctcacccctgtaatccccagcactttgggaggccaagatgggaggatcacttcag

SEQ ID NO: 16434 - RNA, 6306 nt, Homo sapiens
  source 1..6306: mol_type = other RNA
gtccacttctgcctgccctgcctgtgccaaaggtcagcccgggactctgatgacactgatcctccctgaaagccctcccagtctctgcacaaatccagggaaggcatcagaggacaatgtgcagcttcttaggtggcctctccagcatcactagctgggtatccaggactgggctgctcagctccaccaggtgcaaggcccgtgcagggcatcctgagccatgatgcatctcacttttgcatctctgttgccaactcaaggtttctgaaaaacctgacacttccaggggacatcgatgcatcttagctccccgaaatgaagcacacatctctcctggcctaggcaggaccttgaaggaccctctctgcagggaaggcctggctgggcagggcagcctgtcctgtttgcagcatcagggaatgaagcaggctaaagccagcacctgagacctgctctgcccactcctatgcaaccgctgcctcgtggtggtgtgttttggaccctgcctctggcctgctccgaaagagccccattgaacagaggaagggaactgacttcagtattgccaagagtgtttgggcaccgggagtgggaagagggtgaacacactgcaggacccactttttcaacagatgccactagaaaaagcccaaagtgagcagctggcctggggcctgggccttcccaggggcgagggaacacgctgcagtcccagggctatcggcgaactccacgctttcagacgcagccacgagaaccttacgggcaaaccagggacccccgcttgtactgactataccaggtggaaggctgctctttgggccagcgggccattttactcccttcggacttcttgtcagggaagacgcatgtcgaccccccggctgtgaagttgcagtaaaccttgaaggaatccctggagcatccttggttaggatcgacccagtattcaccatctgggaagtcggggtggcagagctgcaggtccttgcaggtgcgggcggggttctgctgcgtgcccaggggccgtttcatctgctcaatctccagcttcagagagttgagagagccgaagatctcttccatgccgtccgcgtagtccacgtagttctcgccattcccgtcgtccagcagctggctggcgtcgatgttccgccgcgtcctggatgcctggattggcaggggctggatgacctctcccggggggcccggggggcctgggggtcctgggtggcctgcctcacccttcgggccagttggacccgaggagcccttagcaccttttggaccaggcggacccggcaggccagggggcccaggaggcccaatcgggccagaaggaccagtgataccctgttctcccttaggaccggaggagccctgggggccagggagaccacggtcgcccttctcaccctgttcacccggaggaccgatgagcccgatcaggcctggatgacccttttcacctttgggaccagaatctcctttgaggccgggaagtcctgggggacccatggggccggggggaccgtccgggcctggggatcctgggagaccttgttctcccacagggccagggatccctcgaaggccatccggtccgggcttcccaggggccccctgggggccgatggggccagtcttcccaggagggccttccaagccggcttctcccttggcccctttctctccctgtctgccttcggggcctgcggggcctgggggacccctttttcctggaggccccgatggacctggttcaccagtagggccgggggatcccgtctgcccgggttcaccatcatctcctttgtcaccagggggaccatcttgacccgcggggccaggctctccgggggggccaggatctccaggaaaacccactgggccagggctgcctttgggaccatcatctccgggagggcctttgggtccagggggtccggcagcacctgaagggcctgactcgcccttctctcccctttctcctttgggtcccggggggccgccttctcccggaaggccaggctcacctgcttcgccaggctcgcccttctctcccactgcaccagggtttcctattccacctgggggaccttgtgggccatcagcacctggagctccggagggtcctcgggggccagggggacccggggggcccatctggcccacgtctcctgtctcacccttctcgcctggaggtcctggcaaaccctgcagccccactggcccagggggtccaggaaagcctctgggaccttcatcacctttctgcccgaaaaggccctgctggccccgaggccccggctcgccgtcagctccagaggggcctggctgtccgatggggccttgaggacctgtaggcccaggaggaccctgttctcctttgtcccccttgcttcctttctgccccggctccccgatctctcccttatctccgtcttctccagggggacccacagggccagctggacccgggagccccacaggcccctggagaccgtctcggccagctgggccttgtgggcctttctcgccaggagcccctttctctcctgccggccctgggggtccctggggcccaggtctccctggaattccgatgggcccagcggctccagctggacctctctcccctggagatcccgcagggcctggtgggccagggggcccttcattgcctttcagtccaagagctcccactggaccaggaagccctcggtccccagggaaaccacgtaatcctggagggccatctttcccagggaggcctgcagggcctgggtcacccttcgtcccttcttttccagcaaggcccggaagcccctgttcaccggggggtccagggggcccagggtggccacgctcacccattgggcccgtttctcccgtgggaccctgagggccgaccacgccgggggggcctggagggccggtcttgccttggaaaccagtctcgcctctctgtccagggtgtcctgggagtccatccttgcctggagggccaggggggccctttggtccaggaaatcctgtgggtccttggggtccattgggtccccgttcaccaggagggccagctgggccgtcacctccggagttgcccttggggccaggcttcccagtgatgccccgggggcctctttcacccctcggacccgttgggcctcgctgcccccgcggtcctggctttccaggggtccccctgccgcccttctctccattggcgccaggaaatccagggaatccaatagagccctttggtccttgtcttcctggataccctggtaaccctgggactccgagttttcccttctccccagggggtcccagaggaccggggtcaccattgggacctccgcgaccctttgggccttcagggccatcttctcccctgggaccgggtgggccgatctccccccgatcacccttgatgcccatgtctcctttaaacccaggaaagccgtcttcacccttctcgccctttgtgcccttcagaccacggatgccatcggcccccttgactcctcgaggacctgggtagccaatcggaccctgggggccaggtggaccctgacctcctttctctcctggagggccttctttgccagggtgtcccgggggtccgtcagcaccgggcattcctggaaggcctggtttccccaagggacccttttctcctggaggaccaattgcaccctgggggcctggaagaccctgggcgcctggattaccctgctgtcctggggggccaggctctccctggggacccacatttccttttggccccggctggccgtccatacccgtgacaccgggaggtccgggaggacctgggggccccttcggcccaagcagaccacgtggcccgggctccccaggcagccccctgggcccaacttctccgtcgtcacccctttctccatcgtctcccggaggtcctggtgggccggaaggaccagggtcacccctgtggcccttctcgcctggcaacccagccaggccgtcgaaaccccggtcacccttggggccagtttgtccaggcattcctctggctccatcactcccagcccgaccccgtcttccgggcttcccggccggaccaggcgggccttgcacacctcgaggaccctgaggccccacgtctcccggctcgcccttcaaacctccgctcccagggggacccacagggccaggtctccctgtgagacccatcgggccagctggtcccctcagtgccaacctggcctgctggagaatggcttgcgcctgggactcctgggctgagaccatggggcctttggagcccgcatcgccgccacctccaaaccggaagggcagcatgagcatggttcctggaggaccgggcaggccatcggccccaggaaggcctgggcgtccaggggggcccctttctccagggtccccgacttggccagtgggacccatggttcctggaggtccgggaagacccgcggggccttctgggccaggcgggccctcgatgagcatgcccggctcgataatcgctggttctcccttttggcctttctcgccccgaggtcctccaatcccttcatagatggtatcctggttcgccggcattcccggcccgatctccgacggggagctggtggggtcgtagtaggggtcgtagtagttctcgtcaaggttccggatcgtttcctcagtgaactccccctccaagtcatccgcaccttcccctggaggcggagctggattggaggagttggaggtgtcggcggtgctggtgggaatttcggccccagcgcctgggtctgtgggctggtcggggttctcctccccctcgccataggtgaggtcatcatacggtgagggcgtgtagtagtcctcactgggcacgtagtcatagtccccgatgccgacgtcctcttccttcccagccccttcactggtttcaggcatgggagcagcttccgtgggggtcggggtcagctcctcggggacctctgtggtttctttggcagcttccacgggcttcttgctgggggtgggctccttccctaggtcttcggggtcttcgtagtaggggtattcgtagtaataggtctcaccctcgccgtctccttccgtgtaatattcatctggattggggtcctgcgactgtggggtgtcaggtactgcggtgtcacagtcagggctgtagtgctcacagtaatcataagctgcccggtggtccgagacaaagagcagctgctggatgtcaccctcaaacacctcctcatccaggatccgggtgccaaacacgatgatgccattgatgtcgatcatggggtggtcgctgcggtcgaggaatttggtggtcttctttttacagtcgaggatcaaggtgacatttttcttgtggacgctgagagcaattctgtgccacttgccatctgacaggttgatgccccggaagagggggtagtcttccgggccaggcttccccgtgtggtcctcgtagaggaagacgggagagcggcccagctccagcccaatctgctggataccctgctcgttgtagatggagaccaggaaggcctggctgcctttcttggctttcacagttgttaggatggagaagtcctcgggaaatgcagacgcagggtacagctgcttggtgggtgcgctgagctgcgcgtctttggtgactctgtaagcgacatccgggcctttggaagatcgccgcgtggcgcaaaagcctgttgtctttgttattccatcaggcaagttgtgaaaatctagaaccttcaggagatctgctggctgagctgcgcggctcggaggcggcgcccacagcagcagcagcagcagcgggggcagcagcggggcgcccgggcggagcgcgctgcgcgctttccagcgggtatggacgtccatgccggcggggcgcgggccggggcgcacaggggcgctcggaggcgcgcggggacgcacaggggcgcgggtcacggcccgggcagcgcactcagcagggaccgcaccactttaggaggtcatggggacctcggcaccccccgttcttctttgtggcggcggctgttctggaaggggcggctggcgcgctcgcccacgggcgggagggctcgactttggcccgcggggcggccgggaccccgctgggctagctcgccctcgcctcctcctcctcctcctccaactccttctcgcctcctcctcgccgccgccgccccgcgacccgctccccgtgggcgctccgctcgagtgaggtcctgcgccagccgcggggacggagagtgcggacctcgccttcggcgc

SEQ ID NO: 16435 - RNA, 6437 nt, Homo sapiens
  source 1..6437: mol_type = other RNA
gtccacttctgcctgccctgcctgtgccaaaggtcagcccgggactctgatgacactgatcctccctgaaagccctcccagtctctgcacaaatccagggaaggcatcagaggacaatgtgcagcttcttaggtggcctctccagcatcactagctgggtatccaggactgggctgctcagctccaccaggtgcaaggcccgtgcagggcatcctgagccatgatgcatctcacttttgcatctctgttgccaactcaaggtttctgaaaaacctgacacttccaggggacatcgatgcatcttagctccccgaaatgaagcacacatctctcctggcctaggcaggaccttgaaggaccctctctgcagggaaggcctggctgggcagggcagcctgtcctgtttgcagcatcagggaatgaagcaggctaaagccagcacctgagacctgctctgcccactcctatgcaaccgctgcctcgtggtggtgtgttttggaccctgcctctggcctgctccgaaagagccccattgaacagaggaagggaactgacttcagtattgccaagagtgtttgggcaccgggagtgggaagagggtgaacacactgcaggacccactttttcaacagatgccactagaaaaagcccaaagtgagcagctggcctggggcctgggccttcccaggggcgagggaacacgctgcagtcccagggctatcggcgaactccacgctttcagacgcagccacgagaaccttacgggcaaaccagggacccccgcttgtactgactataccaggtggaaggctgctctttgggccagcgggccattttactctgtaagatacgagatgggcgggtttaaagtgacaaccgcaaagacgccagaggccaccttaccagtttcccacgcttgaattcactgaaccaggagcccgggttttctttgggccaagaagtgattctggccccttcggacttcttgtcagggaagacgcatgtcgaccccccggctgtgaagttgcagtaaaccttgaaggaatccctggagcatccttggttaggatcgacccagtattcaccatctgggaagtcggggtggcagagctgcaggtccttgcaggtgcgggcggggttctgctgcgtgcccaggggccgtttcatctgctcaatctccagcttcagagagttgagagagccgaagatctcttccatgccgtccgcgtagtccacgtagttctcgccattcccgtcgtccagcagctggctggcgtcgatgttccgccgcgtcctggatgcctggattggcaggggctggatgacctctcccggggggcccggggggcctgggggtcctgggtggcctgcctcacccttcgggccagttggacccgaggagcccttagcaccttttggaccaggcggacccggcaggccagggggcccaggaggcccaatcgggccagaaggaccagtgataccctgttctcccttaggaccggaggagccctgggggccagggagaccacggtcgcccttctcaccctgttcacccggaggaccgatgagcccgatcaggcctggatgacccttttcacctttgggaccagaatctcctttgaggccgggaagtcctgggggacccatggggccggggggaccgtccgggcctggggatcctgggagaccttgttctcccacagggccagggatccctcgaaggccatccggtccgggcttcccaggggccccctgggggccgatggggccagtcttcccaggagggccttccaagccggcttctcccttggcccctttctctccctgtctgccttcggggcctgcggggcctgggggacccctttttcctggaggccccgatggacctggttcaccagtagggccgggggatcccgtctgcccgggttcaccatcatctcctttgtcaccagggggaccatcttgacccgcggggccaggctctccgggggggccaggatctccaggaaaacccactgggccagggctgcctttgggaccatcatctccgggagggcctttgggtccagggggtccggcagcacctgaagggcctgactcgcccttctctcccctttctcctttgggtcccggggggccgccttctcccggaaggccaggctcacctgcttcgccaggctcgcccttctctcccactgcaccagggtttcctattccacctgggggaccttgtgggccatcagcacctggagctccggagggtcctcgggggccagggggacccggggggcccatctggcccacgtctcctgtctcacccttctcgcctggaggtcctggcaaaccctgcagccccactggcccagggggtccaggaaagcctctgggaccttcatcacctttctgcccgaaaaggccctgctggccccgaggccccggctcgccgtcagctccagaggggcctggctgtccgatggggccttgaggacctgtaggcccaggaggaccctgttctcctttgtcccccttgcttcctttctgccccggctccccgatctctcccttatctccgtcttctccagggggacccacagggccagctggacccgggagccccacaggcccctggagaccgtctcggccagctgggccttgtgggcctttctcgccaggagcccctttctctcctgccggccctgggggtccctggggcccaggtctccctggaattccgatgggcccagcggctccagctggacctctctcccctggagatcccgcagggcctggtgggccagggggcccttcattgcctttcagtccaagagctcccactggaccaggaagccctcggtccccagggaaaccacgtaatcctggagggccatctttcccagggaggcctgcagggcctgggtcacccttcgtcccttcttttccagcaaggcccggaagcccctgttcaccggggggtccagggggcccagggtggccacgctcacccattgggcccgtttctcccgtgggaccctgagggccgaccacgccgggggggcctggagggccggtcttgccttggaaaccagtctcgcctctctgtccagggtgtcctgggagtccatccttgcctggagggccaggggggccctttggtccaggaaatcctgtgggtccttggggtccattgggtccccgttcaccaggagggccagctgggccgtcacctccggagttgcccttggggccaggcttcccagtgatgccccgggggcctctttcacccctcggacccgttgggcctcgctgcccccgcggtcctggctttccaggggtccccctgccgcccttctctccattggcgccaggaaatccagggaatccaatagagccctttggtccttgtcttcctggataccctggtaaccctgggactccgagttttcccttctccccagggggtcccagaggaccggggtcaccattgggacctccgcgaccctttgggccttcagggccatcttctcccctgggaccgggtgggccgatctccccccgatcacccttgatgcccatgtctcctttaaacccaggaaagccgtcttcacccttctcgccctttgtgcccttcagaccacggatgccatcggcccccttgactcctcgaggacctgggtagccaatcggaccctgggggccaggtggaccctgacctcctttctctcctggagggccttctttgccagggtgtcccgggggtccgtcagcaccgggcattcctggaaggcctggtttccccaagggacccttttctcctggaggaccaattgcaccctgggggcctggaagaccctgggcgcctggattaccctgctgtcctggggggccaggctctccctggggacccacatttccttttggccccggctggccgtccatacccgtgacaccgggaggtccgggaggacctgggggccccttcggcccaagcagaccacgtggcccgggctccccaggcagccccctgggcccaacttctccgtcgtcacccctttctccatcgtctcccggaggtcctggtgggccggaaggaccagggtcacccctgtggcccttctcgcctggcaacccagccaggccgtcgaaaccccggtcacccttggggccagtttgtccaggcattcctctggctccatcactcccagcccgaccccgtcttccgggcttcccggccggaccaggcgggccttgcacacctcgaggaccctgaggccccacgtctcccggctcgcccttcaaacctccgctcccagggggacccacagggccaggtctccctgtgagacccatcgggccagctggtcccctcagtgccaacctggcctgctggagaatggcttgcgcctgggactcctgggctgagaccatggggcctttggagcccgcatcgccgccacctccaaaccggaagggcagcatgagcatggttcctggaggaccgggcaggccatcggccccaggaaggcctgggcgtccaggggggcccctttctccagggtccccgacttggccagtgggacccatggttcctggaggtccgggaagacccgcggggccttctgggccaggcgggccctcgatgagcatgcccggctcgataatcgctggttctcccttttggcctttctcgccccgaggtcctccaatcccttcatagatggtatcctggttcgccggcattcccggcccgatctccgacggggagctggtggggtcgtagtaggggtcgtagtagttctcgtcaaggttccggatcgtttcctcagtgaactccccctccaagtcatccgcaccttcccctggaggcggagctggattggaggagttggaggtgtcggcggtgctggtgggaatttcggccccagcgcctgggtctgtgggctggtcggggttctcctccccctcgccataggtgaggtcatcatacggtgagggcgtgtagtagtcctcactgggcacgtagtcatagtccccgatgccgacgtcctcttccttcccagccccttcactggtttcaggcatgggagcagcttccgtgggggtcggggtcagctcctcggggacctctgtggtttctttggcagcttccacgggcttcttgctgggggtgggctccttccctaggtcttcggggtcttcgtagtaggggtattcgtagtaataggtctcaccctcgccgtctccttccgtgtaatattcatctggattggggtcctgcgactgtggggtgtcaggtactgcggtgtcacagtcagggctgtagtgctcacagtaatcataagctgcccggtggtccgagacaaagagcagctgctggatgtcaccctcaaacacctcctcatccaggatccgggtgccaaacacgatgatgccattgatgtcgatcatggggtggtcgctgcggtcgaggaatttggtggtcttctttttacagtcgaggatcaaggtgacatttttcttgtggacgctgagagcaattctgtgccacttgccatctgacaggttgatgccccggaagagggggtagtcttccgggccaggcttccccgtgtggtcctcgtagaggaagacgggagagcggcccagctccagcccaatctgctggataccctgctcgttgtagatggagaccaggaaggcctggctgcctttcttggctttcacagttgttaggatggagaagtcctcgggaaatgcagacgcagggtacagctgcttggtgggtgcgctgagctgcgcgtctttggtgactctgtaagcgacatccgggcctttggaagatcgccgcgtggcgcaaaagcctgttgtctttgttattccatcaggcaagttgtgaaaatctagaaccttcaggagatctgctggctgagctgcgcggctcggaggcggcgcccacagcagcagcagcagcagcgggggcagcagcggggcgcccgggcggagcgcgctgcgcgctttccagcgggtatggacgtccatgccggcggggcgcgggccggggcgcacaggggcgctcggaggcgcgcggggacgcacaggggcgcgggtcacggcccgggcagcgcactcagcagggaccgcaccactttaggaggtcatggggacctcggcaccccccgttcttctttgtggcggcggctgttctggaaggggcggctggcgcgctcgcccacgggcgggagggctcgactttggcccgcggggcggccgggaccccgctgggctagctcgccctcgcctcctcctcctcctcctccaactccttctcgcctcctcctcgccgccgccgccccgcgacccgctccccgtgggcgctccgctcgagtgaggtcctgcgccagccgcggggacggagagtgcggacctcgccttcggcg

SEQ ID NO: 16436 - RNA, 5227 nt, Homo sapiens
  source 1..5227: mol_type = other RNA
gtccagttttcccaggaatccctgcggttctcatcaacatacattcgaaacaggatcctcaaacaacaggccaggctgctggtttcttgttttagaagattgggtttagacttgcccttaaaacctgctcgccacaggacagtccgctgctcgtaattggagttgaaggcctttgagaatgaatgggattcctgcaaacagtccaacagcttgaagaggtgctgggaagacatgtacttatacatgccctgatcctccgtctctatgtggatatctgcatccagcgtgtcttgctgggcggcaaccatgtgctctgcatcctcctttttgctcgtcgcagggtagaacacaatgttgtcaatggtctgtatcaattccaactggaccacacacttgatgaggaggctggcaaacagtttctgatttgcgtatggtctacccttccagctgtcatctgttgggttagagagctggctctgtcccctctcagagggatttttatctatgctgcttaaagactggcggtccagatccacatccaaatgcttttctgatgaatcttcctccattcctacaggtctccatgtcagcaaaacatgtgggatggttgttttgaaaatatccaacatacagttgcaggtttcatcccagacttcaggactgaatttctctccattggatattactaagttttctaagcaatttgtacctgatcgcgccaactgttcattatcttgtttgacacaccactgcaattgtgcaaatacatcagaaagaagaacttcattcaaagcttcataaaactgggtaaaaacatcacaaatagcataaagtgcgtgattgcaggttgttgtcatccactcagatttctctgacagttgctcagggagtttcatattgtcaaaaatccgaaacacgattctgaacaggtcctgccaccagtgcttttcaaaggtgtggccatagctcttcatgatctcaaacatgactgtgagtccccttgttcgtacatctaacttgcatctattaatgatgcaggagagttcgaataagatggggaaccagcctcggacccagactctgtcaccaggagctacattcatgtcatcacttgtgtattcttgtagcacccgaggcctctcagagacgtatttgccacagaagcggatgagccgaatcgcttccatgctcgtgtcagggaaagcggcgttgcaggcgaactctgataagcacttcacagcatcctgaaaggaatcgatggctgcaggaaaatggtgctggaaaatagttgtgacaatgtggcaagtggtctggaaggccagctccacaatgttcccatcatgatcagaggctgcctggtggaacacggcaaagatgttcttccaacctgagcggatgttggccgcctgggagttcaccatctgggcaatgcagcggatcgccatgtcccggatggtgggagacctgtttttcttcataatatgctcaaagggcctcagaaaatctttctggaaacggaagttggctaattcacccttctcaagaaacttcatggagagttgccttaatgagtcaacagcaaagatagccacatcttcattagggttgcagccaaccttattgaagtgatctccaatcacatgccatattcgagaccactgtagtcggatccgattcatgttgtagtatgatatctccacaatcttctgcaagctgaacatgcgaggatggtggggggaagccagttcatccatggacacagcacacagccagcggacaaagtcaactattgcatttccatccagtctggtagacccagtaaaaatcctgtccacagctacaaccacactctgcgagctggtctcaccaaccgattcttggaagctggccatctgtcttttatccactccgccactcaccaaattaccgaggccaaggcccatgaactcttctcctgccaatgtgtggcccttcaggctcccttctctttcacgcccagatccagacaggtagcgcgtcttcacaccggttcctatcagctgagcgagctccagctggctgatgcatttcaagatctcatgccaggaattcccaaggtagttgccatcggtgtgagccactgtgataagcgtcttaatggtgtcgatgtttttctgcttcatttctgtgatgctggagctggctgtgagtagggagaagcgagcaagagcctgaacataggcatctcgttccagctgcattccaaagatgcaggcgattcggattgcacatcggatgccttccaaacacaaggaggccacttcagtgtcatcacagttctggagtccgatgctgtaggctgccaatagtggcgtccacaccagtttgaacattggccggacatggtccaggtgagtggcactggtaaacggggctttggcatggctcacagcctccatcagagctttggctgttttagccatttgctccatctctaagttgtacagcagccgccgctgcttttcactagctacattctgcttagtagatttggttgcaatcgttagctcttttgtttctttcattgcaattttcttgccttctatctcttcatagatgcttgagagatactcttctggcagatctttactatcattgataccccgattcattttaatatactgctctttcgtcattttattttttacctgaggactgtgcaagtctgtagtcagcataataattgaatacgctaggacataagcagtgtcagcactagcaaacagagtttgcccttggttgcattctatgtatcttgcggcaaacttctccattaatcggtcaatcttttgggcttctccaggtaggcggaaaccttctaggaatgtccgcagggctgagacaaattctttttcacagaagtcaagttggtccacgtaggcatacatcacctccttgttgaaccttgcgctatctcccagaaaatcgcctacttgggtggaatccaggcgctcctcctggtgcaggaattgggctatgtcttcaactgacgttcccagcatgccctgctcctggagaaactggatccccctcttgggtttcttgttgaacagctcgatgccgtgttcaatgatttctttttgttgcttgatgacctcaaattgctcagggtcatcctgaacagttgtctgggtccccgaggacactgtggactccatggacgtcacactacaccgtcttgccatgtcaaggcctttcccatcccctatttcctgatccgtgagcctctcctgaccgaggctggtctggtggttgggattcacatacaggtctttgctccactccaccatgcacttgagaatggacacgaggcactccaggcctttcttcctcaggctgagctcctgcagaggtgtcattcccagctcatgtccacttcttccctgagcaattttggataaatcatttacaaggcgctcaaaaatgttagcagcatttaaatcacagtcgtagttgacataaatatccacaacacactgggcatctgcacagatcctcgtcagagtctgaatgaccatccacctgtgctcaaaagaacttgttgatgtttctaaaatgttcaggaaaatctctttgaaaaagacctctatctgcattttcaagtgcattttaaagtttgaaagaagagtaagaaaaatggcaagagagagctcaaagacatcaggcactgaagagacgccgtttttggacaaggccacacagagatattgcttgattgcattgatgaacatctcgtgagtcctgaatacggggccagcattttgcaacacagagaggagcagctgcagggaaaccaccttggaacgcagctcatgggattttgggtctggagggccttcaccaaggggtttcatggacagcttgcacagggagcggaacacaaggaaggcatccttctgcagaacgtgggagaacctggcagccacttgatgtccttgtgcatccgattccagattatctgctgacgacaaggactgcctgtcatcggctatcccgttggtctgtgagttttcatcaactcctgggggaatagcacattcctggcactccagttcacctagaactctctcaggttctgtcagaccatgcttttccgctgcttctttaatggcagatgtgactacatcttccaagatgtccttcaccacctcctgggctccgtcatcagtccctgacagtgatgagcctctttctctgggtgcgtctccattttctgtgcttacttttccagaatcactcctggcatgttcaccgttggttaaatctgttttttcgggagttgttggtttgctttgtgcctgactgtgcttcaaacgaacgaactttggggatactgctgcagcttggatcacaggggactggggttttgactggattggtttttccagttctctggcctcctgcaacacttggttttccatgcgggtgaaaatgacgttcagcatctgagtaagggtagccttggcagtggtttgattgatgagatttttgctggccaaatagatattgtaacatgttctcactgtctgcaggatagtaccctcatgaatttcaatgtgtggggaagtcactgcagtcagaagagccttaattatttgtaactgaaccccttcatcagtctgagggccctgaaaacaactgcaaatggtttcaacaattctgtcgatcagccgcttcccaggggctccactgtcaggggcgttgccagtgatgtgcccgtatgcgatgagtttctgcaagcagtcaagggatgtgctgactacccttggggacttggactggcaagctagctcgaatggaagaaaatacttgtcagcttcaatgaagtttgcctttggtggtgcagcagtgccaagcctctgcttttctatttctgctttaatttcatcgagcgccacctggcaggccctgcgcagctgggagtgctggggccgcttcacctccttgtcggctaggatcttctccagggcccgggacacgaacatgctcttggtctggctctcctgcatggccccggcccggcgggggctgacggccccgcgggcgggcggcgtgagcgagatggcgagctaggctgcgggcccggcgtcccggccggcaccggccgcgtccgtccgcgccgccccgtcaggaagcgacacctcggccccacggcgccgccatgttggagcgcgtcacgtgaccacgt

SEQ ID NO: 16437 - RNA, 5214 nt, Homo sapiens
  source 1..5214: mol_type = other RNA
gtccagttttcccaggaatccctgcggttctcatcaacatacattcgaaacaggatcctcaaacaacaggccaggctgctggtttcttgttttagaagattgggtttagacttgcccttaaaacctgctcgccacaggacagtccgctgctcgtaattggagttgaaggcctttgagaatgaatgggattcctgcaaacagtccaacagcttgaagaggtgctgggaagacatgtacttatacatgccctgatcctccgtctctatgtggatatctgcatccagcgtgtcttgctgggcggcaaccatgtgctctgcatcctcctttttgctcgtcgcagggtagaacacaatgttgtcaatggtctgtatcaattccaactggaccacacacttgatgaggaggctggcaaacagtttctgatttgcgtatggtctacccttccagctgtcatctgttgggttagagagctggctctgtcccctctcagagggatttttatctatgctgcttaaagactggcggtccagatccacatccaaatgcttttctgatgaatcttcctccattcctacaggtctccatgtcagcaaaacatgtgggatggttgttttgaaaatatccaacatacagttgcaggtttcatcccagacttcaggactgaatttctctccattggatattactaagttttctaagcaatttgtacctgatcgcgccaactgttcattatcttgtttgacacaccactgcaattgtgcaaatacatcagaaagaagaacttcattcaaagcttcataaaactgggtaaaaacatcacaaatagcataaagtgcgtgattgcaggttgttgtcatccactcagatttctctgacagttgctcagggagtttcatattgtcaaaaatccgaaacacgattctgaacaggtcctgccaccagtgcttttcaaaggtgtggccatagctcttcatgatctcaaacatgactgtgagtccccttgttcgtacatctaacttgcatctattaatgatgcaggagagttcgaataagatggggaaccagcctcggacccagactctgtcaccaggagctacattcatgtcatcacttgtgtattcttgtagcacccgaggcctctcagagacgtatttgccacagaagcggatgagccgaatcgcttccatgctcgtgtcagggaaagcggcgttgcaggcgaactctgataagcacttcacagcatcctgaaaggaatcgatggctgcaggaaaatggtgctggaaaatagttgtgacaatgtggcaagtggtctggaaggccagctccacaatgttcccatcatgatcagaggctgcctggtggaacacggcaaagatgttcttccaacctgagcggatgttggccgcctgggagttcaccatctgggcaatgcagcggatcgccatgtcccggatggtgggagacctgtttttcttcataatatgctcaaagggcctcagaaaatctttctggaaacggaagttggctaattcacccttctcaagaaacttcatggagagttgccttaatgagtcaacagcaaagatagccacatcttcattagggttgcagccaaccttattgaagtgatctccaatcacatgccatattcgagaccactgtagtcggatccgattcatgttgtagtatgatatctccacaatcttctgcaagctgaacatgcgaggatggtggggggaagccagttcatccatggacacagcacacagccagcggacaaagtcaactattgcatttccatccagtctggtagacccagtaaaaatcctgtccacagctacaaccacactctgcgagctggtctcaccaaccgattcttggaagctggccatctgtcttttatccactccgccactcaccaaattaccgaggccaaggcccatgaactcttctcctgccaatgtgtggcccttcaggctcccttctctttcacgcccagatccagacaggtagcgcgtcttcacaccggttcctatcagctgagcgagctccagctggctgatgcatttcaagatctcatgccaggaattcccaaggtagttgccatcggtgtgagccactgtgataagcgtcttaatggtgtcgatgtttttctgcttcatttctgtgatgctggagctggctgtgagtagggagaagcgagcaagagcctgaacataggcatctcgttccagctgcattccaaagatgcaggcgattcggattgcacatcggatgccttccaaacacaaggaggccacttcagtgtcatcacagttctggagtccgatgctgtaggctgccaatagtggcgtccacaccagtttgaacattggccggacatggtccaggtgagtggcactggtaaacggggctttggcatggctcacagcctccatcagagctttggctgttttagccatttgctccatctctaagttgtacagcagccgccgctgcttttcactagctacattctgcttagtagatttggttgcaatcgttagctcttttgtttctttcattgcaattttcttgccttctatctcttcatagatgcttgagagatactcttctggcagatctttactatcattgataccccgattcattttaatatactgctctttcgtcattttattttttacctgaggactgtgcaagtctgtagtcagcataataattgaatacgctaggacataagcagtgtcagcactagcaaacagagtttgcccttggttgcattctatgtatcttgcggcaaacttctccattaatcggtcaatcttttgggcttctccaggtaggcggaaaccttctaggaatgtccgcagggctgagacaaattctttttcacagaagtcaagttggtccacgtaggcatacatcacctccttgttgaaccttgcgctatctcccagaaaatcgcctacttgggtggaatccaggcgctcctcctggtgcaggaattgggctatgtcttcaactgacgttcccagcatgccctgctcctggagaaactggatccccctcttgggtttcttgttgaacagctcgatgccgtgttcaatgatttctttttgttgcttgatgacctcaaattgctcagggtcatcctgaacagttgtctgggtccccgaggacactgtggactccatggacgtcacactacaccgtcttgccatgtcaaggcctttcccatcccctatttcctgatccgtgagcctctcctgaccgaggctggtctggtggttgggattcacatacaggtctttgctccactccaccatgcacttgagaatggacacgaggcactccaggcctttcttcctcaggctgagctcctgcagaggtgtcattcccagctcatgtccacttcttccctgagcaattttggataaatcatttacaaggcgctcaaaaatgttagcagcatttaaatcacagtcgtagttgacataaatatccacaacacactgggcatctgcacagatcctcgtcagagtctgaatgaccatccacctgtgctcaaaagaacttgttgatgtttctaaaatgttcaggaaaatctctttgaaaaagacctctatctgcattttcaagtgcattttaaagtttgaaagaagagtaagaaaaatggcaagagagagctcaaagacatcaggcactgaagagacgccgtttttggacaaggccacacagagatattgcttgattgcattgatgaacatctcgtgagtcctgaatacggggccagcattttgcaacacagagaggagcagctgcagggaaaccaccttggaacgcagctcatgggattttgggtctggagggccttcaccaaggggtttcatggacagcttgcacagggagcggaacacaaggaaggcatccttctgcagaacgtgggagaacctggcagccacttgatgtccttgtgcatccgattccagattatctgctgacgacaaggactgcctgtcatcggctatcccgttggtctgtgagttttcatcaactcctgggggaatagcacattcctggcactccagttcacctagaactctctcaggttctgtcagaccatgcttttccgctgctttaatggcagatgtgactacatcttccaagatgtccttcaccacctcctgggctccgtcatcagtccctgacagtgatgagcctctttctctgggtgcgtctccattttctgtgcttacttttccagaatcactcctggcatgttcaccgttggttaaatctgttttttcgggagttgttggtttgctttgtgcctgactgtgcttcaaacgaacgaactttggggatactgctgcagcttggatcacaggggactggggttttgactggattggtttttccagttctctggcctcctgcaacacttggttttccatgcgggtgaaaatgacgttcagcatctgagtaagggtagccttggcagtggtttgattgatgagatttttgctggccaaatagatattgtaacatgttctcactgtctgcaggatagtaccctcatgaatttcaatgtgtggggaagtcactgcagtcagaagagccttaattatttgtaactgaaccccttcatcagtctgagggccctgaaaacaactgcaaatggtttcaacaattctgtcgatcagccgcttcccaggggctccactgtcaggggcgttgccagtgatgtgcccgtatgcgatgagtttctgcaagcagtcaagggatgtgctgactacccttggggacttggactggcaagctagctcgaatggaagaaaatacttgtcagcttcaatgaagtttgcctttggtggtgcagcagtgccaagcctctgcttttctatttctgctttaatttcatcgagcgccacctggcaggccctgcgcagctgggagtgctggggccgcttcacctccttgtcggctaggatcttctccagggcccgggacacgaacatgctcttggtctggctctcctgcatggccccggcccggcgggggctgacggccccgcgggcgggcggcgtgagcgagatggcgagctaggctgcgggcccggcgtcccggccggcaccggccgcgtccgtccgcgccgccccgtcaggaagcgacacctcggccccacggcgccgccatgttggagcgcgtcac

SEQ ID NO: 16438 - RNA, 347 nt, Homo sapiens
  source 1..347: mol_type = other RNA
gtccagttttcccaggaatccctgggtctcccttctctccgaactcaccatggtctccagccagccctggaagccctttctctccttttatccctggggtcccaggttggccatcggggccaggtgtcccagggatacccgggatgccagggatggctgggggcccggtgcagctgagctgggcctgggagatatcgattaggcccaggagcaggagcaacatcagtactgggatgctgccccatgggatcttcatcatcatactgtgtcagacgcctcctgggaagctggtgtcctgtgaggccactgggctgagcagcagtgggaccaggagccgagagcctact

SEQ ID NO: 16439 - RNA, 500 nt, Homo sapiens
  source 1..500: mol_type = other RNA
gtccagttttcccaggaatccctgggtctcccttctctccgaactcaccatggtctccagccagccctggaagccctttctctccttttatccctggggtcccaggttggccatcggggccaggtgtcccagggatacccgggatgccagggatggctgggggcccggtgcagctgagctgggcctgggagatatcgattaggcccaggagcaggagcaacatcagtactgggatgctgccccatgggatcttcatcatcatactgtgtcagacgcctcctttccatctccttcggtccagcagtccctttccgcaacatggagtcaggcccacttgactttaaagccccatctgctaccggctgcataacctcaggcaagtgccttaacctctctgagcctcttggcaatgctgatttcaacctgacagggctgggaagctggtgtcctgtgaggccactgggctgagcagcagtgggaccaggagccgagagcctact

SEQ ID NO: 16440 - RNA, 1001 nt, Homo sapiens
  source 1..1001: mol_type = other RNA
gtccagttttcccaggaatccctttgtaaagaccttttcctctctgtaaccatggtggtgctgctactgaccagcagagggcagtgttgcaccaacattctctatggctctgcattgcttttgcctgaccttggacgggaacattgaaatcattaattagtggtcagtgtcatcatctttttcaaaaggccttattttatcctcagtgcatagtcagaacaaggtcttgccacagtgtacagatgaggaagcagagcctcagaaacataagaaacttaattactggtaattttggtcacaccacgtcctaaatttagactctcagaatggtatgaacccattgctgtgtgtctgagcagcaaagcattgataatccattacctgctttatgcatcatgaagcactttctgatcctcaatatcagacaattctcatcttattctcctccagtttgtaaatgagcaaactgtggcttctagaggctatatcatttgacttacagcttttttttttttagagaggcccaggctggcctcgaactcctggcttcaggtgatcctcccacctcagcctcccaagtagctgggattacaggtgtgagccattgcacctggcaccagcatattcacaatcagttccatcttagagactgtttggtggactcccaaaaatattagtttaaaaatgacagagcctggcgttttgcaatttttatgtgatgaaatgtactgagttctcatataaatattgctccttgttttgcaaaaggaattaggcccctttccctgtctcagcagctgcaccggttattagcaatcccctagggaactggaatagctttagatcaacagtggttctcaaaagggactatcaaatgacacacctgtccccagctccagattccgatatccacaccccaaacatccaatcactgtttctcatagtcttttgatgttttttgtttttgttgtttttggtttttggtatttttttgagacaaa

SEQ ID NO: 16441 - RNA, 70 nt, Homo sapiens
  source 1..70: mol_type = other RNA
gtccctctccaaatgtgtcttgatcccccaccccaagacacatttggagagggaccctcccaactcagat

SEQ ID NO: 16442 - RNA, 133 nt, Homo sapiens
  source 1..133: mol_type = other RNA
gtccctctccaaatgtgtcttgatcccccaccccaagacacatttggagagggaccctcccaactcagataaactgtggagagtgtaggagataggaaatggactgagaacttcctggtcccaccagagaagc

SEQ ID NO: 16443 - RNA, 66 nt, Homo sapiens
  source 1..66: mol_type = other RNA
gtccctctccaaatgtgtcttggggtgggggatcaagacacatttggagagggaacctcccaactc

SEQ ID NO: 16444 - RNA, 4638 nt, Homo sapiens
  source 1..4638: mol_type = other RNA
gtcctaggaggctcctctgtggccaggcttctgcctccctgcaccctgagggaccattcgggtgcctcagggatgcccttccctcccaggggcactgacagcactggctgaaaggtctgaagagccagaggaggagccctgctggctggcccaggatggggcaaggagggagggaaagccaggggatggggagggacatgagatggagtttaaggcacacagcgagcgatggaggagggaggtgctggcctctcccctctgaattaactcccccaggagctcagctctggcctcagtttggtgaggttcagaagactcccagcaataaaaagtatttcttggatgatcaagtcctcccttactccagcctcctcttctcagctccccaggtggtgtgggaggggcccagtggcctggggtggggggtaaggggcgacgggatgacagagactgctgctgctctcaggcgggcaagggaggccctgatggcgccagtaccgcggggcagagcaccagctgcggggctgctaaggcgtcacctgcgtacctttccgggcctgctgaaaagctcacaccatcctccatgcatcagaaggggaagcggaaagtgaaaggatcctcccccgagtctactctgcattctgcccacccagctgcttgcccccattccagggcccctgcaggacaggccaccccaggaggcctccactcatttgagatttcagaagattcagggaccctggagcttagggagggggagcacccaccacttccttggtctgctgatgaggtctctgctgctctctccctggaggggagtgggtggaaggtcaagaggggagagatggaagtaaaagcagaaaacaaaaccaaaccagaaaaccaccggtttgtaaattggcaacaagacctgcctgctggctgccctgaggcccacgggtctgctcccacagaggaaggaggcaggaagcggctggcaggctccagctcccgcccggccccgctgagggctggccagcctcatggctccgaggccgggactcctgccatgcgcctaacaggtccaaggtcctctccggtctgggagctgccctctgcgcccctcgagcattctcctggatcccggcgtctgctcctaggtcttctcttcccggtctgtttttctccttgttatgttcctgggtttaattttcagagacagttcccatagggcctcctcagccaggtggtcactgaagtcattgaagaagtttataatgtcgtcgttcctccgcatgtcatagtgcgcctgctggaagcagcgcatgctgtcgaggatgttgaactgctgccaccgcttggagaagttcactttcccgtcgatgtagtctgggtttcccaggtgaacgaaggtcaggtcctgcaggatcagccccaggtacgggatgcacggcggttccacctccgagagggcggcccggtaggctcggaaggaggacgagctgtcgatcagtgtgcagtactcggccaggccctctgaagtctgcttctgccactccagcctgcggatgggcgccgagtccagggcagagaggatggccaagtaggagttgaagttattcagcttccgcaagtgcttcatgatcttgatgaacttcaagagcagccgttccctgtcctgggccttttcctgtaacatgattatggaccggacccagtaggacatgttgttgaagtgctccgtgaactgggtcaagttggggctcttctcctcattctgctcttttgcccaaagcaaaacctcaggaatctctattttatagaagagctcagcatccagcagcgttagctgctccgctatctcatggctgtgaaagtcgtgcaaggtccccggcctggctgctaccccccgggctgccaggggctggctggaggtggcacacctgagtagcttcttctggtccaccttgtccaggatgttcttccggagcacacgggccaggctcagctccccattgcacaccaggcggaagaccagttccatcagcagcttcaggatctcttctgtcaactccaccaggcagagctcatccaccacccgtaccagcacgaagaacgtgttcttgctgacgcgcttcttgaatgtgtcggcaaagggagagaatttctcatatctgtactgcagcttcttgatgagctcctctggggagatgaaggtcctgtaggtggtcaggaatgcctcgcagtacaacaccaaatctttcctgtcagtctcagtagcatggaccagtaagatgtccccagatcctccgcggacgtccggcccgtcatcaccctcctgcttgagcgtcagcctggacataatttcgttgtggtcaatgagggacagctcgtccacttcctcctccgactgagccgactccagagcatctggtgactttggggccctctcactgccgtctctgctgtccttcccagggacgccgctgaccgctgagggatctctgggatgtccgtctttcccagccggtggctccagctgccgctgcttggggggtagggcgggcggcggggccagctcctgcacggagtccaccccactgaaggagtcgctgaagccgtatacctccatgaggagcttgttcttctgctggtagatgtgctcgttctgtggcgtctggtagaacatagagggctgcggctccgagtagtcctccagcaactgcatgtaggccagcatgtgtttgtttttcttctctggtagaggaggtggtttttctgggtcaccggttgactcaggagcagtaaaatcacccacaaattcgacaggggctgaggaacctccatgctgaaagggcagaatagcagcaaagggcgcgtaggggacggatgggatcggggctgtgctctgcaggtcctccccagagatgttgtcatactgcgagggatgccgctcgtaggacaccctgcagccagagccgtccgccgtctgggaggctgcgctcctgcgcttcttctcggggagagcaggtggcgtatctgtctgctgccctggggccagaggtccgtctggctggggatggccgccaagaggcagctggaaaggagggccaagaaatggagacccagactcccccaaagactctggcaacgggctaaggttccaggccgtctgctgaggtatctggtctgcgttagagaggtcttgctggaggaattcatagtcgggatcatagtggtctagtgtttcacagcttgtgttccgggagcactgcccactgtccctgtccagagaggacagctgctcgtctgacttgctgagcttgcctatgctgctgcagggggagaggcggggcgactctccaccatatgagtggctgcctcctgacagtcgcctctgtgcgtaacagtcaacatcaaaatcctgcctattgattccaacaggcaaactggagccactggtggctcggctcatgggggccaccacagccactcgggtaggggacggcgccgactgtcttttcttgggtggcaatgctggtggaggactattatcaaccacccgaatgccaggcagaggaggcttggggggcgcgacctcttcatccgtggcatctgggaggagctcagttgactgtgacatcccagtcgtcttgtttaggatctctacctcgcggtctgtcagggggagctctgctgggccatcaggcttgctggcaggggaactgggcttcacggggctcgtcggagacggacgtccctgcttctcgatggtgagcctgaccagctccttcactccatccagcacagccttgatgacccccttcacagtcgtcaccatctccttgtcttctgagttcacgccttccagcatcacttggtcagaccagcgaatgaggttggcgaggctttggtacactcggctatagcaggaagagagggctgagctgtgctgaattcgaggatcgttctgcaccaggggtaagatggcctccagcaccttgctggctgaccctggaagcatctccagtaccttcttatcaattgccattttgtccacaatggtcttaaagtagcgcagggcactgacaacttccttctctttctcctccagccagctcaggttcttctgcctttgagacctggaagccacagcactggtggacataaattctactgcctgctgctccagatccaaggggagagggtagccctctggtagaaatctgtctgttgcctcctggaagagaggaaacctggattctttgttcacaggcttctctggaatctttacggacacctcagctggttttcccttctttgatggcgttctcttgattttgggtgagtggaatttgtccatcagcttcatggtgaaggaagagagatgagaacgctgagagtctggaacgacacctcctgtcctcttgttctgttccaaggttgtcaggctgggacgaaatcccaagaaagaaatgggcatgtggtcactatcatagcagactgccagttagggacatcagaatatatttctctgtcctcaagttaggaagtgagaggacaaacctggccttctgtgttgtttcagccactaattggttttgtcaattaggcaaaacataatttctctaagcctcttttctcatccacaggcattag

SEQ ID NO: 16445 - RNA, 4666 nt, Homo sapiens
  source 1..4666: mol_type = other RNA
gtcctaggaggctcctctgtggccaggcttctgcctccctgcaccctgagggaccattcgggtgcctcagggatgcccttccctcccaggggcactgacagcactggctgaaaggtctgaagagccagaggaggagccctgctggctggcccaggatggggcaaggagggagggaaagccaggggatggggagggacatgagatggagtttaaggcacacagcgagcgatggaggagggaggtgctggcctctcccctctgaattaactcccccaggagctcagctctggcctcagtttggtgaggttcagaagactcccagcaataaaaagtatttcttggatgatcaagtcctcccttactccagcctcctcttctcagctccccaggtggtgtgggaggggcccagtggcctggggtggggggtaaggggcgacgggatgacagagactgctgctgctctcaggcgggcaagggaggccctgatggcgccagtaccgcggggcagagcaccagctgcggggctgctaaggcgtcacctgcgtacctttccgggcctgctgaaaagctcacaccatcctccatgcatcagaaggggaagcggaaagtgaaaggatcctcccccgagtctactctgcattctgcccacccagctgcttgcccccattccagggcccctgcaggacaggccaccccaggaggcctccactcatttgagatttcagaagattcagggaccctggagcttagggagggggagcacccaccacttccttggtctgctgatgaggtctctgctgctctctccctggaggggagtgggtggaaggtcaagaggggagagatggaagtaaaagcagaaaacaaaaccaaaccagaaaaccaccggtttgtaaattggcaacaagacctgcctgctggctgccctgaggcccacgggtctgctcccacagaggaaggaggcaggaagcggctggcaggctccagctcccgcccggccccgctgagggctggccagcctcatggctccgaggccgggactcctgccatgcgcctaacaggtccaaggtcctctccggtctgggagctgccctctgcgcccctcgagcattctcctggatcccggcgtctgctcctaggtcttctcttcccggtctgtttttctccttgttatgttcctgggtttaattttcagagacagttcccatagggcctcctcagccaggtggtcactgaagtcattgaagaagtttataatgtcgtcgttcctccgcatgtcatagtgcgcctgctggaagcagcgcatgctgtcgaggatgttgaactgctgccaccgcttggagaagttcactttcccgtcgatgtagtctgggtttcccaggtgaacgaaggtcaggtcctgcaggatcagccccaggtacgggatgcacggcggttccacctccgagagggcggcccggtaggctcggaaggaggacgagctgtcgatcagtgtgcagtactcggccaggccctctgaagtctgcttctgccactccagcctgcggatgggcgccgagtccagggcagagaggatggccaagtaggagttgaagttattcagcttccgcaagtgcttcatgatcttgatgaacttcaagagcagccgttccctgtcctgggccttttcctgtaacatgattatggaccggacccagtaggacatgttgttgaagtgctccgtgaactgggtcaagttggggctcttctcctcattctgctcttttgcccaaagcaaaacctcaggaatctctattttatagaagagctcagcatccagcagcgttagctgctccgctatctcatggctgtgaaagtcgtgcaaggtccccggcctggctgctaccccccgggctgccaggggctggctggaggtggcacacctgagtagcttcttctggtccaccttgtccaggatgttcttccggagcacacgggccaggctcagctccccattgcacaccaggcggaagaccagttccatcagcagcttcaggatctcttctgtcaactccaccaggcagagctcatccaccacccgtaccagcacgaagaacgtgttcttgctgacgcgcttcttgaatgtgtcggcaaagggagagaatttctcatatctgtactgcagcttcttgatgagctcctctggggagatgaaggtcctgtaggtggtcaggaatgcctcgcagtacaacaccaaatctttcctgtcagtctcagtagcatggaccagtaagatgtccccagatcctccgcggacgtccggcccgtcatcaccctcctgcttgagcgtcagcctggacataatttcgttgtggtcaatgagggacagctcgtccacttcctcctccgactgagccgactccagagcatctggtgactttggggccctctcactgccgtctctgctgtccttcccagggacgccgctgaccgctgagggatctctgggatgtccgtctttcccagccggtggctccagctgccgctgcttggggggtagggcgggcggcggggccagctcctgcacggagtccaccccactgaaggagtcgctgaagccgtatacctccatgaggagcttgttcttctgctggtagatgtgctcgttctgtggcgtctggtagaacatagagggctgcggctccgagtagtcctccagcaactgcatgtaggccagcatgtgtttgtttttcttctctggtagaggaggtggtttttctgggtcaccggttgactcaggagcagtaaaatcacccacaaattcgacaggggctgaggaacctccatgctgaaagggcagaatagcagcaaagggcgcgtaggggacggatgggatcggggctgtgctctgcaggtcctccccagagatgttgtcatactgcgagggatgccgctcgtaggacaccctgcagccagagccgtccgccgtctgggaggctgcgctcctgcgcttcttctcggggagagcaggtggcgtatctgtctgctgccctggggccagaggtccgtctggctggggatggccgccaagaggcagctggaaaggagggccaagaaatggagacccagactcccccaaagactctggcaacgggctaaggttccaggccgtctgctgaggtatctggtctgcgttagagaggtcttgctggaggaattcatagtcgggatcatagtggtctagtgtttcacagcttgtgttccgggagcactgcccactgtccctgtccagagaggacagctgctcgtctgacttgctgagcttgcctatgctgctgcagggggagaggcggggcgactctccaccatatgagtggctgcctcctgacagtcgcctctgtgcgtaacagtcaacatcaaaatcctgcctattgattccaacaggcaaactggagccactggtggctcggctcatgggggccaccacagccactcgggtaggggacggcgccgactgtcttttcttgggtggcaatgctggtggaggactattatcaaccacccgaatgccaggcagaggaggcttggggggcgcgacctcttcatccgtggcatctgggaggagctcagttgactgtgacatcccagtcgtcttgtttaggatctctacctcgcggtctgtcagggggagctctgctgggccatcaggcttgctggcaggggaactgggcttcacggggctcgtcggagacggacgtccctgcttctcgatggtgagcctgaccagctccttcactccatccagcacagccttgatgacccccttcacagtcgtcaccatctccttgtcttctgagttcacgccttccagcatcacttggtcagaccagcgaatgaggttggcgaggctttggtacactcggctatagcaggaagagagggctgagctgtgctgaattcgaggatcgttctgcaccaggggtaagatggcctccagcaccttgctggctgaccctggaagcatctccagtaccttcttatcaattgccattttgtccacaatggtcttaaagtagcgcagggcactgacaacttccttctctttctcctccagccagctcaggttcttctgcctttgagacctggaagccacagcactggtggacataaattctactgcctgctgctccagatccaaggggagagggtagccctctggtagaaatctgtctgttgcctctttgttcacaggcttctctggaatctttacggacacctcagctggttttcccttctttgatggcgttctcttgattttgggtgagtggaatttgtccatcagcttcatggtgaaggaagagagatgagaacgctgagagtctgctttctcgatcttgccggacatttccgggctgcgccggaggccgaggccgccgctcatcgggcccgggccgggccgccgcggggcgacaggggcggcgcgcccgccgctcgcctcggccctggctcgccacgcctcagacccgcgccggcatggcgggctccgcgcggccgcggccctgcgctcggcgaccgcgctccagcccgcccgggcccagccgctcccgccgcgcccgccgccgccgctccgcctcccgcgcgcccgccgccgctcccccggcccgcgagccggccgcagcgcagcgac

SEQ ID NO: 16446 - RNA, 4620 nt, Homo sapiens
  source 1..4620: mol_type = other RNA
gtcctaggaggctcctctgtggccaggcttctgcctccctgcaccctgagggaccattcgggtgcctcagggatgcccttccctcccaggggcactgacagcactggctgaaaggtctgaagagccagaggaggagccctgctggctggcccaggatggggcaaggagggagggaaagccaggggatggggagggacatgagatggagtttaaggcacacagcgagcgatggaggagggaggtgctggcctctcccctctgaattaactcccccaggagctcagctctggcctcagtttggtgaggttcagaagactcccagcaataaaaagtatttcttggatgatcaagtcctcccttactccagcctcctcttctcagctccccaggtggtgtgggaggggcccagtggcctggggtggggggtaaggggcgacgggatgacagagactgctgctgctctcaggcgggcaagggaggccctgatggcgccagtaccgcggggcagagcaccagctgcggggctgctaaggcgtcacctgcgtacctttccgggcctgctgaaaagctcacaccatcctccatgcatcagaaggggaagcggaaagtgaaaggatcctcccccgagtctactctgcattctgcccacccagctgcttgcccccattccagggcccctgcaggacaggccaccccaggaggcctccactcatttgagatttcagaagattcagggaccctggagcttagggagggggagcacccaccacttccttggtctgctgatgaggtctctgctgctctctccctggaggggagtgggtggaaggtcaagaggggagagatggaagtaaaagcagaaaacaaaaccaaaccagaaaaccaccggtttgtaaattggcaacaagacctgcctgctggctgccctgaggcccacgggtctgctcccacagaggaaggaggcaggaagcggctggcaggctccagctcccgcccggccccgctgagggctggccagcctcatggctccgaggccgggactcctgccatgcgcctaacaggtccaaggtcctctccggtctgggagctgccctctgcgcccctcgagcattctcctggatcccggcgtctgctcctaggtcttctcttcccggtctgtttttctccttgttatgttcctgggtttaattttcagagacagttcccatagggcctcctcagccaggtggtcactgaagtcattgaagaagtttataatgtcgtcgttcctccgcatgtcatagtgcgcctgctggaagcagcgcatgctgtcgaggatgttgaactgctgccaccgcttggagaagttcactttcccgtcgatgtagtctgggtttcccaggtgaacgaaggtcaggtcctgcaggatcagccccaggtacgggatgcacggcggttccacctccgagagggcggcccggtaggctcggaaggaggacgagctgtcgatcagtgtgcagtactcggccaggccctctgaagtctgcttctgccactccagcctgcggatgggcgccgagtccagggcagagaggatggccaagtaggagttgaagttattcagcttccgcaagtgcttcatgatcttgatgaacttcaagagcagccgttccctgtcctgggccttttcctgtaacatgattatggaccggacccagtaggacatgttgttgaagtgctccgtgaactgggtcaagttggggctcttctcctcattctgctcttttgcccaaagcaaaacctcaggaatctctattttatagaagagctcagcatccagcagcgttagctgctccgctatctcatggctgtgaaagtcgtgcaaggtccccggcctggctgctaccccccgggctgccaggggctggctggaggtggcacacctgagtagcttcttctggtccaccttgtccaggatgttcttccggagcacacgggccaggctcagctccccattgcacaccaggcggaagaccagttccatcagcagcttcaggatctcttctgtcaactccaccaggcagagctcatccaccacccgtaccagcacgaagaacgtgttcttgctgacgcgcttcttgaatgtgtcggcaaagggagagaatttctcatatctgtactgcagcttcttgatgagctcctctggggagatgaaggtcctgtaggtggtcaggaatgcctcgcagtacaacaccaaatctttcctgtcagtctcagtagcatggaccagtaagatgtccccagatcctccgcggacgtccggcccgtcatcaccctcctgcttgagcgtcagcctggacataatttcgttgtggtcaatgagggacagctcgtccacttcctcctccgactgagccgactccagagcatctggtgactttggggccctctcactgccgtctctgctgtccttcccagggacgccgctgaccgctgagggatctctgggatgtccgtctttcccagccggtggctccagctgccgctgcttggggggtagggcgggcggcggggccagctcctgcacggagtccaccccactgaaggagtcgctgaagccgtatacctccatgaggagcttgttcttctgctggtagatgtgctcgttctgtggcgtctggtagaacatagagggctgcggctccgagtagtcctccagcaactgcatgtaggccagcatgtgtttgtttttcttctctggtagaggaggtggtttttctgggtcaccggttgactcaggagcagtaaaatcacccacaaattcgacaggggctgaggaacctccatgctgaaagggcagaatagcagcaaagggcgcgtaggggacggatgggatcggggctgtgctctgcaggtcctccccagagatgttgtcatactgcgagggatgccgctcgtaggacaccctgcagccagagccgtccgccgtctgggaggctgcgctcctgcgcttcttctcggggagagcaggtggcgtatctgtctgctgccctggggccagaggtccgtctggctggggatggccgccaagaggcagctggaaaggagggccaagaaatggagacccagactcccccaaagactctggcaacgggctaaggttccaggccgtctgctgaggtatctggtctgcgttagagaggtcttgctggaggaattcatagtcgggatcatagtggtctagtgtttcacagcttgtgttccgggagcactgcccactgtccctgtccagagaggacagctgctcgtctgacttgctgagcttgcctatgctgctgcagggggagaggcggggcgactctccaccatatgagtggctgcctcctgacagtcgcctctgtgcgtaacagtcaacatcaaaatcctgcctattgattccaacaggcaaactggagccactggtggctcggctcatgggggccaccacagccactcgggtaggggacggcgccgactgtcttttcttgggtggcaatgctggtggaggactattatcaaccacccgaatgccaggcagaggaggcttggggggcgcgacctcttcatccgtggcatctgggaggagctcagttgactgtgacatcccagtcgtcttgtttaggatctctacctcgcggtctgtcagggggagctctgctgggccatcaggcttgctggcaggggaactgggcttcacggggctcgtcggagacggacgtccctgcttctcgatggtgagcctgaccagctccttcactccatccagcacagccttgatgacccccttcacagtcgtcaccatctccttgtcttctgagttcacgccttccagcatcacttggtcagaccagcgaatgaggttggcgaggctttggtacactcggctatagcaggaagagagggctgagctgtgctgaattcgaggatcgttctgcaccaggggtaagatggcctccagcaccttgctggctgaccctggaagcatctccagtaccttcttatcaattgccattttgtccacaatggtcttaaagtagcgcagggcactgacaacttccttctctttctcctccagccagctcaggttcttctgcctttgagacctggaagccacagcactggtggacataaattctactgcctgctgctccagatccaaggggagagggtagccctctggtagaaatctgtctgttgcctctttgttcacaggcttctctggaatctttacggacacctcagctggttttcccttctttgatggcgttctcttgattttgggtgagtggaatttgtccatcagcttcatggtgaaggaagagagatgagaacgctgagagtctggaacgacacctcctgtcctcttgttctgttccaaggttgtcaggctgggacgaaatcccaagaaagaaatgggcatgtggtcactatcatagcagactgccagttagggacatcagaatatatttctctgtcctcaagttaggaagtgagaggacaaacctggccttctgtgttgtttcagccactaattggttttgtcaattaggcaaaacataatttctctaagcctcttttctcatccacaggcattagcctagt

SEQ ID NO: 16447 - RNA, 4402 nt, Homo sapiens
  source 1..4402: mol_type = other RNA
gtcctaggaggctcctctgtggccaggcttctgcctccctgcaccctgagggaccattcgggtgcctcagggatgcccttccctcccaggggcactgacagcactggctgaaaggtctgaagagccagaggaggagccctgctggctggcccaggatggggcaaggagggagggaaagccaggggatggggagggacatgagatggagtttaaggcacacagcgagcgatggaggagggaggtgctggcctctcccctctgaattaactcccccaggagctcagctctggcctcagtttggtgaggttcagaagactcccagcaataaaaagtatttcttggatgatcaagtcctcccttactccagcctcctcttctcagctccccaggtggtgtgggaggggcccagtggcctggggtggggggtaaggggcgacgggatgacagagactgctgctgctctcaggcgggcaagggaggccctgatggcgccagtaccgcggggcagagcaccagctgcggggctgctaaggcgtcacctgcgtacctttccgggcctgctgaaaagctcacaccatcctccatgcatcagaaggggaagcggaaagtgaaaggatcctcccccgagtctactctgcattctgcccacccagctgcttgcccccattccagggcccctgcaggacaggccaccccaggaggcctccactcatttgagatttcagaagattcagggaccctggagcttagggagggggagcacccaccacttccttggtctgctgatgaggtctctgctgctctctccctggaggggagtgggtggaaggtcaagaggggagagatggaagtaaaagcagaaaacaaaaccaaaccagaaaaccaccggtttgtaaattggcaacaagacctgcctgctggctgccctgaggcccacgggtctgctcccacagaggaaggaggcaggaagcggctggcaggctccagctcccgcccggccccgctgagggctggccagcctcatggctccgaggccgggactcctgccatgcgcctaacaggtccaaggtcctctccggtctgggagctgccctctgcgcccctcgagcattctcctggatcccggcgtctgctcctaggtcttctcttcccggtctgtttttctccttgttatgttcctgggtttaattttcagagacagttcccatagggcctcctcagccaggtggtcactgaagtcattgaagaagtttataatgtcgtcgttcctccgcatgtcatagtgcgcctgctggaagcagcgcatgctgtcgaggatgttgaactgctgccaccgcttggagaagttcactttcccgtcgatgtagtctgggtttcccaggtgaacgaaggtcaggtcctgcaggatcagccccaggtacgggatgcacggcggttccacctccgagagggcggcccggtaggctcggaaggaggacgagctgtcgatcagtgtgcagtactcggccaggccctctgaagtctgcttctgccactccagcctgcggatgggcgccgagtccagggcagagaggatggccaagtaggagttgaagttattcagcttccgcaagtgcttcatgatcttgatgaacttcaagagcagccgttccctgtcctgggccttttcctgtaacatgattatggaccggacccagtaggacatgttgttgaagtgctccgtgaactgggtcaagttggggctcttctcctcattctgctcttttgcccaaagcaaaacctcaggaatctctattttatagaagagctcagcatccagcagcgttagctgctccgctatctcatggctgtgaaagtcgtgcaaggtccccggcctggctgctaccccccgggctgccaggggctggctggaggtggcacacctgagtagcttcttctggtccaccttgtccaggatgttcttccggagcacacgggccaggctcagctccccattgcacaccaggcggaagaccagttccatcagcagcttcaggatctcttctgtcaactccaccaggcagagctcatccaccacccgtaccagcacgaagaacgtgttcttgctgacgcgcttcttgaatgtgtcggcaaagggagagaatttctcatatctgtactgcagcttcttgatgagctcctctggggagatgaaggtcctgtaggtggtcaggaatgcctcgcagtacaacaccaaatctttcctgtcagtctcagtagcatggaccagtaagatgtccccagatcctccgcggacgtccggcccgtcatcaccctcctgcttgagcgtcagcctggacataatttcgttgtggtcaatgagggacagctcgtccacttcctcctccgactgagccgactccagagcatctggtgactttggggccctctcactgccgtctctgctgtccttcccagggacgccgctgaccgctgagggatctctgggatgtccgtctttcccagccggtggctccagctgccgctgcttggggggtagggcgggcggcggggccagctcctgcacggagtccaccccactgaaggagtcgctgaagccgtatacctccatgaggagcttgttcttctgctggtagatgtgctcgttctgtggcgtctggtagaacatagagggctgcggctccgagtagtcctccagcaactgcatgtaggccagcatgtgtttgtttttcttctctggtagaggaggtggtttttctgggtcaccggttgactcaggagcagtaaaatcacccacaaattcgacaggggctgaggaacctccatgctgaaagggcagaatagcagcaaagggcgcgtaggggacggatgggatcggggctgtgctctgcaggtcctccccagagatgttgtcatactgcgagggatgccgctcgtaggacaccctgcagccagagccgtccgccgtctgggaggctgcgctcctgcgcttcttctcggggagagcaggtggcgtatctgtctgctgccctggggccagaggtccgtctggctggggatggccgccaagaggcagctggaaaggagggccaagaaatggagacccagactcccccaaagactctggcaacgggctaaggttccaggccgtctgctgaggtatctggtctgcgttagagaggtcttgctggaggaattcatagtcgggatcatagtggtctagtgtttcacagcttgtgttccgggagcactgcccactgtccctgtccagagaggacagctgctcgtctgacttgctgagcttgcctatgctgctgcagggggagaggcggggcgactctccaccatatgagtggctgcctcctgacagtcgcctctgtgcgtaacagtcaacatcaaaatcctgcctattgattccaacaggcaaactggagccactggtggctcggctcatgggggccaccacagccactcgggtaggggacggcgccgactgtcttttcttgggtggcaatgctggtggaggactattatcaaccacccgaatgccaggcagaggaggcttggggggcgcgacctcttcatccgtggcatctgggaggagctcagttgactgtgacatcccagtcgtcttgtttaggatctctacctcgcggtctgtcagggggagctctgctgggccatcaggcttgctggcaggggaactgggcttcacggggctcgtcggagacggacgtccctgcttctcgatggtgagcctgaccagctccttcactccatccagcacagccttgatgacccccttcacagtcgtcaccatctccttgtcttctgagttcacgccttccagcatcacttggtcagaccagcgaatgaggttggcgaggctttggtacactcggctatagcaggaagagagggctgagctgtgctgaattcgaggatcgttctgcaccaggggtaagatggcctccagcaccttgctggctgaccctggaagcatctccagtaccttcttatcaattgccattttgtccacaatggtcttaaagtagcgcagggcactgacaacttccttctctttctcctccagccagctcaggttcttctgcctttgagacctggaagccacagcactggtggacataaattctactgcctgctgctccagatccaaggggagagggtagccctctggtagaaatctgtctgttgcctctttgttcacaggcttctctggaatctttacggacacctcagctggttttcccttctttgatggcgttctcttgattttgggtgagtggaatttgtccatcagcttcatggtgaaggaagagagatgagaacgctgagagtctgtgtccatggcagcacggtcgctcggtctggcagcctgggt

SEQ ID NO: 16448 - RNA, 4582 nt, Homo sapiens
  source 1..4582: mol_type = other RNA
gtcctaggaggctcctctgtggccaggcttctgcctccctgcaccctgagggaccattcgggtgcctcagggatgcccttccctcccaggggcactgacagcactggctgaaaggtctgaagagccagaggaggagccctgctggctggcccaggatggggcaaggagggagggaaagccaggggatggggagggacatgagatggagtttaaggcacacagcgagcgatggaggagggaggtgctggcctctcccctctgaattaactcccccaggagctcagctctggcctcagtttggtgaggttcagaagactcccagcaataaaaagtatttcttggatgatcaagtcctcccttactccagcctcctcttctcagctccccaggtggtgtgggaggggcccagtggcctggggtggggggtaaggggcgacgggatgacagagactgctgctgctctcaggcgggcaagggaggccctgatggcgccagtaccgcggggcagagcaccagctgcggggctgctaaggcgtcacctgcgtacctttccgggcctgctgaaaagctcacaccatcctccatgcatcagaaggggaagcggaaagtgaaaggatcctcccccgagtctactctgcattctgcccacccagctgcttgcccccattccagggcccctgcaggacaggccaccccaggaggcctccactcatttgagatttcagaagattcagggaccctggagcttagggagggggagcacccaccacttccttggtctgctgatgaggtctctgctgctctctccctggaggggagtgggtggaaggtcaagaggggagagatggaagtaaaagcagaaaacaaaaccaaaccagaaaaccaccggtttgtaaattggcaacaagacctgcctgctggctgccctgaggcccacgggtctgctcccacagaggaaggaggcaggaagcggctggcaggctccagctcccgcccggccccgctgagggctggccagcctcatggctccgaggccgggactcctgccatgcgcctaacaggtccaaggtcctctccggtctgggagctgccctctgcgcccctcgagcattctcctggatcccggcgtctgctcctaggtcttctcttcccggtctgtttttctccttgttatgttcctgggtttaattttcagagacagttcccatagggcctcctcagccaggtggtcactgaagtcattgaagaagtttataatgtcgtcgttcctccgcatgtcatagtgcgcctgctggaagcagcgcatgctgtcgaggatgttgaactgctgccaccgcttggagaagttcactttcccgtcgatgtagtctgggtttcccaggtgaacgaaggtcaggtcctgcaggatcagccccaggtacgggatgcacggcggttccacctccgagagggcggcccggtaggctcggaaggaggacgagctgtcgatcagtgtgcagtactcggccaggccctctgaagtctgcttctgccactccagcctgcggatgggcgccgagtccagggcagagaggatggccaagtaggagttgaagttattcagcttccgcaagtgcttcatgatcttgatgaacttcaagagcagccgttccctgtcctgggccttttcctgtaacatgattatggaccggacccagtaggacatgttgttgaagtgctccgtgaactgggtcaagttggggctcttctcctcattctgctcttttgcccaaagcaaaacctcaggaatctctattttatagaagagctcagcatccagcagcgttagctgctccgctatctcatggctgtgaaagtcgtgcaaggtccccggcctggctgctaccccccgggctgccaggggctggctggaggtggcacacctgagtagcttcttctggtccaccttgtccaggatgttcttccggagcacacgggccaggctcagctccccattgcacaccaggcggaagaccagttccatcagcagcttcaggatctcttctgtcaactccaccaggcagagctcatccaccacccgtaccagcacgaagaacgtgttcttgctgacgcgcttcttgaatgtgtcggcaaagggagagaatttctcatatctgtactgcagcttcttgatgagctcctctggggagatgaaggtcctgtaggtggtcaggaatgcctcgcagtacaacaccaaatctttcctgtcagtctcagtagcatggaccagtaagatgtccccagatcctccgcggacgtccggcccgtcatcaccctcctgcttgagcgtcagcctggacataatttcgttgtggtcaatgagggacagctcgtccacttcctcctccgactgagccgactccagagcatctggtgactttggggccctctcactgccgtctctgctgtccttcccagggacgccgctgaccgctgagggatctctgggatgtccgtctttcccagccggtggctccagctgccgctgcttggggggtagggcgggcggcggggccagctcctgcacggagtccaccccactgaaggagtcgctgaagccgtatacctccatgaggagcttgttcttctgctggtagatgtgctcgttctgtggcgtctggtagaacatagagggctgcggctccgagtagtcctccagcaactgcatgtaggccagcatgtgtttgtttttcttctctggtagaggaggtggtttttctgggtcaccggttgactcaggagcagtaaaatcacccacaaattcgacaggggctgaggaacctccatgctgaaagggcagaatagcagcaaagggcgcgtaggggacggatgggatcggggctgtgctctgcaggtcctccccagagatgttgtcatactgcgagggatgccgctcgtaggacaccctgcagccagagccgtccgccgtctgggaggctgcgctcctgcgcttcttctcggggagagcaggtggcgtatctgtctgctgccctggggccagaggtccgtctggctggggatggccgccaagaggcagctggaaaggagggccaagaaatggagacccagactcccccaaagactctggcaacgggctaaggttccaggccgtctgctgaggtatctggtctgcgttagagaggtcttgctggaggaattcatagtcgggatcatagtggtctagtgtttcacagcttgtgttccgggagcactgcccactgtccctgtccagagaggacagctgctcgtctgacttgctgagcttgcctatgctgctgcagggggagaggcggggcgactctccaccatatgagtggctgcctcctgacagtcgcctctgtgcgtaacagtcaacatcaaaatcctgcctattgattccaacaggcaaactggagccactggtggctcggctcatgggggccaccacagccactcgggtaggggacggcgccgactgtcttttcttgggtggcaatgctggtggaggactattatcaaccacccgaatgccaggcagaggaggcttggggggcgcgacctcttcatccgtggcatctgggaggagctcagttgactgtgacatcccagtcgtcttgtttaggatctctacctcgcggtctgtcagggggagctctgctgggccatcaggcttgctggcaggggaactgggcttcacggggctcgtcggagacggacgtccctgcttctcgatggtgagcctgaccagctccttcactccatccagcacagccttgatgacccccttcacagtcgtcaccatctccttgtcttctgagttcacgccttccagcatcacttggtcagaccagcgaatgaggttggcgaggctttggtacactcggctatagcaggaagagagggctgagctgtgctgaattcgaggatcgttctgcaccaggggtaagatggcctccagcaccttgctggctgaccctggaagcatctccagtaccttcttatcaattgccattttgtccacaatggtcttaaagtagcgcagggcactgacaacttccttctctttctcctccagccagctcaggttcttctgcctttgagacctggaagccacagcactggtggacataaattctactgcctgctgctccagatccaaggggagagggtagccctctggtagaaatctgtctgttgcctctttgttcacaggcttctctggaatctttacggacacctcagctggttttcccttctttgatggcgttctcttgattttgggtgagtggaatttgtccatcagcttcatggtgaaggaagagagatgagaacgctgagagtcttgtttccaggggtacagatgacttcgtttcaagggcttctgtttttcaatagcattgcccattttaaagccagaggacacagggcccttcccagccccagcgtctttccggagcagcaactgaggaccgagtcactggctgaaaggggatatctcttggacatcccaaaccacccagcggcagaacccaggcagcctcacaagggaagcctgaggaatctc

SEQ ID NO: 16449 - RNA, 4552 nt, Homo sapiens
  source 1..4552: mol_type = other RNA
gtcctaggaggctcctctgtggccaggcttctgcctccctgcaccctgagggaccattcgggtgcctcagggatgcccttccctcccaggggcactgacagcactggctgaaaggtctgaagagccagaggaggagccctgctggctggcccaggatggggcaaggagggagggaaagccaggggatggggagggacatgagatggagtttaaggcacacagcgagcgatggaggagggaggtgctggcctctcccctctgaattaactcccccaggagctcagctctggcctcagtttggtgaggttcagaagactcccagcaataaaaagtatttcttggatgatcaagtcctcccttactccagcctcctcttctcagctccccaggtggtgtgggaggggcccagtggcctggggtggggggtaaggggcgacgggatgacagagactgctgctgctctcaggcgggcaagggaggccctgatggcgccagtaccgcggggcagagcaccagctgcggggctgctaaggcgtcacctgcgtacctttccgggcctgctgaaaagctcacaccatcctccatgcatcagaaggggaagcggaaagtgaaaggatcctcccccgagtctactctgcattctgcccacccagctgcttgcccccattccagggcccctgcaggacaggccaccccaggaggcctccactcatttgagatttcagaagattcagggaccctggagcttagggagggggagcacccaccacttccttggtctgctgatgaggtctctgctgctctctccctggaggggagtgggtggaaggtcaagaggggagagatggaagtaaaagcagaaaacaaaaccaaaccagaaaaccaccggtttgtaaattggcaacaagacctgcctgctggctgccctgaggcccacgggtctgctcccacagaggaaggaggcaggaagcggctggcaggctccagctcccgcccggccccgctgagggctggccagcctcatggctccgaggccgggactcctgccatgcgcctaacaggtccaaggtcctctccggtctgggagctgccctctgcgcccctcgagcattctcctggatcccggcgtctgctcctaggtcttctcttcccggtctgtttttctccttgttatgttcctgggtttaattttcagagacagttcccatagggcctcctcagccaggtggtcactgaagtcattgaagaagtttataatgtcgtcgttcctccgcatgtcatagtgcgcctgctggaagcagcgcatgctgtcgaggatgttgaactgctgccaccgcttggagaagttcactttcccgtcgatgtagtctgggtttcccaggtgaacgaaggtcaggtcctgcaggatcagccccaggtacgggatgcacggcggttccacctccgagagggcggcccggtaggctcggaaggaggacgagctgtcgatcagtgtgcagtactcggccaggccctctgaagtctgcttctgccactccagcctgcggatgggcgccgagtccagggcagagaggatggccaagtaggagttgaagttattcagcttccgcaagtgcttcatgatcttgatgaacttcaagagcagccgttccctgtcctgggccttttcctgtaacatgattatggaccggacccagtaggacatgttgttgaagtgctccgtgaactgggtcaagttggggctcttctcctcattctgctcttttgcccaaagcaaaacctcaggaatctctattttatagaagagctcagcatccagcagcgttagctgctccgctatctcatggctgtgaaagtcgtgcaaggtccccggcctggctgctaccccccgggctgccaggggctggctggaggtggcacacctgagtagcttcttctggtccaccttgtccaggatgttcttccggagcacacgggccaggctcagctccccattgcacaccaggcggaagaccagttccatcagcagcttcaggatctcttctgtcaactccaccaggcagagctcatccaccacccgtaccagcacgaagaacgtgttcttgctgacgcgcttcttgaatgtgtcggcaaagggagagaatttctcatatctgtactgcagcttcttgatgagctcctctggggagatgaaggtcctgtaggtggtcaggaatgcctcgcagtacaacaccaaatctttcctgtcagtctcagtagcatggaccagtaagatgtccccagatcctccgcggacgtccggcccgtcatcaccctcctgcttgagcgtcagcctggacataatttcgttgtggtcaatgagggacagctcgtccacttcctcctccgactgagccgactccagagcatctggtgactttggggccctctcactgccgtctctgctgtccttcccagggacgccgctgaccgctgagggatctctgggatgtccgtctttcccagccggtggctccagctgccgctgcttggggggtagggcgggcggcggggccagctcctgcacggagtccaccccactgaaggagtcgctgaagccgtatacctccatgaggagcttgttcttctgctggtagatgtgctcgttctgtggcgtctggtagaacatagagggctgcggctccgagtagtcctccagcaactgcatgtaggccagcatgtgtttgtttttcttctctggtagaggaggtggtttttctgggtcaccggttgactcaggagcagtaaaatcacccacaaattcgacaggggctgaggaacctccatgctgaaagggcagaatagcagcaaagggcgcgtaggggacggatgggatcggggctgtgctctgcaggtcctccccagagatgttgtcatactgcgagggatgccgctcgtaggacaccctgcagccagagccgtccgccgtctgggaggctgcgctcctgcgcttcttctcggggagagcaggtggcgtatctgtctgctgccctggggccagaggtccgtctggctggggatggccgccaagaggcagctggaaaggagggccaagaaatggagacccagactcccccaaagactctggcaacgggctaaggttccaggccgtctgctgaggtatctggtctgcgttagagaggtcttgctggaggaattcatagtcgggatcatagtggtctagtgtttcacagcttgtgttccgggagcactgcccactgtccctgtccagagaggacagctgctcgtctgacttgctgagcttgcctatgctgctgcagggggagaggcggggcgactctccaccatatgagtggctgcctcctgacagtcgcctctgtgcgtaacagtcaacatcaaaatcctgcctattgattccaacaggcaaactggagccactggtggctcggctcatgggggccaccacagccactcgggtaggggacggcgccgactgtcttttcttgggtggcaatgctggtggaggactattatcaaccacccgaatgccaggcagaggaggcttggggggcgcgacctcttcatccgtggcatctgggaggagctcagttgactgtgacatcccagtcgtcttgtttaggatctctacctcgcggtctgtcagggggagctctgctgggccatcaggcttgctggcaggggaactgggcttcacggggctcgtcggagacggacgtccctgcttctcgatggtgagcctgaccagctccttcactccatccagcacagccttgatgacccccttcacagtcgtcaccatctccttgtcttctgagttcacgccttccagcatcacttggtcagaccagcgaatgaggttggcgaggctttggtacactcggctatagcaggaagagagggctgagctgtgctgaattcgaggatcgttctgcaccaggggtaagatggcctccagcaccttgctggctgaccctggaagcatctccagtaccttcttatcaattgccattttgtccacaatggtcttaaagtagcgcagggcactgacaacttccttctctttctcctccagccagctcaggtttttgttcacaggcttctctggaatctttacggacacctcagctggttttcccttctttgatggcgttctcttgattttgggtgagtggaatttgtccatcagcttcatggtgaaggaagagagatgagaacgctgagagtctgctttctcgatcttgccggacatttccgggctgcgccggaggccgaggccgccgctcatcgggcccgggccgggccgccgcggggcgacaggggcggcgcgcccgccgctcgcctcggccctggctcgccacgcctcagacccgcgccggcatggcgggctccgcgcggccgcggccctgcgctcggcgaccgcgctccagcccgcccgggcccagccgctcccgccgcgcccgccgccgccgctccgcctcccgcgcgcccgccgccgctcccccggcccgcgagccggccgcagcgcagcgac

SEQ ID NO: 16450 - RNA, 4794 nt, Homo sapiens
  source 1..4794: mol_type = other RNA
gtcctaggaggctcctctgtggccaggcttctgcctccctgcaccctgagggaccattcgggtgcctcagggatgcccttccctcccaggggcactgacagcactggctgaaaggtctgaagagccagaggaggagccctgctggctggcccaggatggggcaaggagggagggaaagccaggggatggggagggacatgagatggagtttaaggcacacagcgagcgatggaggagggaggtgctggcctctcccctctgaattaactcccccaggagctcagctctggcctcagtttggtgaggttcagaagactcccagcaataaaaagtatttcttggatgatcaagtcctcccttactccagcctcctcttctcagctccccaggtggtgtgggaggggcccagtggcctggggtggggggtaaggggcgacgggatgacagagactgctgctgctctcaggcgggcaagggaggccctgatggcgccagtaccgcggggcagagcaccagctgcggggctgctaaggcgtcacctgcgtacctttccgggcctgctgaaaagctcacaccatcctccatgcatcagaaggggaagcggaaagtgaaaggatcctcccccgagtctactctgcattctgcccacccagctgcttgcccccattccagggcccctgcaggacaggccaccccaggaggcctccactcatttgagatttcagaagattcagggaccctggagcttagggagggggagcacccaccacttccttggtctgctgatgaggtctctgctgctctctccctggaggggagtgggtggaaggtcaagaggggagagatggaagtaaaagcagaaaacaaaaccaaaccagaaaaccaccggtttgtaaattggcaacaagacctgcctgctggctgccctgaggcccacgggtctgctcccacagaggaaggaggcaggaagcggctggcaggctccagctcccgcccggccccgctgagggctggccagcctcatggctccgaggccgggactcctgccatgcgcctaacaggtccaaggtcctctccggtctgggagctgccctctgcgcccctcgagcattctcctggatcccggcgtctgctcctaggtcttctcttcccggtctgtttttctccttgttatgttcctgggtttaattttcagagacagttcccatagggcctcctcagccaggtggtcactgaagtcattgaagaagtttataatgtcgtcgttcctccgcatgtcatagtgcgcctgctggaagcagcgcatgctgtcgaggatgttgaactgctgccaccgcttggagaagttcactttcccgtcgatgtagtctgggtttcccaggtgaacgaaggtcaggtcctgcaggatcagccccaggtacgggatgcacggcggttccacctccgagagggcggcccggtaggctcggaaggaggacgagctgtcgatcagtgtgcagtactcggccaggccctctgaagtctgcttctgccactccagcctgcggatgggcgccgagtccagggcagagaggatggccaagtaggagttgaagttattcagcttccgcaagtgcttcatgatcttgatgaacttcaagagcagccgttccctgtcctgggccttttcctgtaacatgattatggaccggacccagtaggacatgttgttgaagtgctccgtgaactgggtcaagttggggctcttctcctcattctgctcttttgcccaaagcaaaacctcaggaatctctattttatagaagagctcagcatccagcagcgttagctgctccgctatctcatggctgtgaaagtcgtgcaaggtccccggcctggctgctaccccccgggctgccaggggctggctggaggtggcacacctgagtagcttcttctggtccaccttgtccaggatgttcttccggagcacacgggccaggctcagctccccattgcacaccaggcggaagaccagttccatcagcagcttcaggatctcttctgtcaactccaccaggcagagctcatccaccacccgtaccagcacgaagaacgtgttcttgctgacgcgcttcttgaatgtgtcggcaaagggagagaatttctcatatctgtactgcagcttcttgatgagctcctctggggagatgaaggtcctgtaggtggtcaggaatgcctcgcagtacaacaccaaatctttcctgtcagtctcagtagcatggaccagtaagatgtccccagatcctccgcggacgtccggcccgtcatcaccctcctgcttgagcgtcagcctggacataatttcgttgtggtcaatgagggacagctcgtccacttcctcctccgactgagccgactccagagcatctggtgactttggggccctctcactgccgtctctgctgtccttcccagggacgccgctgaccgctgagggatctctgggatgtccgtctttcccagccggtggctccgagggcacgggcaagctgccgtgccggctgagaaaggagttagagacggacacactgaggccctgagcggcactgccgtcctcgggggtgaaggccactttagtttgctggacacagtgggagacagaggagaaggaagaagcagcacaggaggccagctgccgctgcttggggggtagggcgggcggcggggccagctcctgcacggagtccaccccactgaaggagtcgctgaagccgtatacctccatgaggagcttgttcttctgctggtagatgtgctcgttctgtggcgtctggtagaacatagagggctgcggctccgagtagtcctccagcaactgcatgtaggccagcatgtgtttgtttttcttctctggtagaggaggtggtttttctgggtcaccggttgactcaggagcagtaaaatcacccacaaattcgacaggggctgaggaacctccatgctgaaagggcagaatagcagcaaagggcgcgtaggggacggatgggatcggggctgtgctctgcaggtcctccccagagatgttgtcatactgcgagggatgccgctcgtaggacaccctgcagccagagccgtccgccgtctgggaggctgcgctcctgcgcttcttctcggggagagcaggtggcgtatctgtctgctgccctggggccagaggtccgtctggctggggatggccgccaagaggcagctggaaaggagggccaagaaatggagacccagactcccccaaagactctggcaacgggctaaggttccaggccgtctgctgaggtatctggtctgcgttagagaggtcttgctggaggaattcatagtcgggatcatagtggtctagtgtttcacagcttgtgttccgggagcactgcccactgtccctgtccagagaggacagctgctcgtctgacttgctgagcttgcctatgctgctgcagggggagaggcggggcgactctccaccatatgagtggctgcctcctgacagtcgcctctgtgcgtaacagtcaacatcaaaatcctgcctattgattccaacaggcaaactggagccactggtggctcggctcatgggggccaccacagccactcgggtaggggacggcgccgactgtcttttcttgggtggcaatgctggtggaggactattatcaaccacccgaatgccaggcagaggaggcttggggggcgcgacctcttcatccgtggcatctgggaggagctcagttgactgtgacatcccagtcgtcttgtttaggatctctacctcgcggtctgtcagggggagctctgctgggccatcaggcttgctggcaggggaactgggcttcacggggctcgtcggagacggacgtccctgcttctcgatggtgagcctgaccagctccttcactccatccagcacagccttgatgacccccttcacagtcgtcaccatctccttgtcttctgagttcacgccttccagcatcacttggtcagaccagcgaatgaggttggcgaggctttggtacactcggctatagcaggaagagagggctgagctgtgctgaattcgaggatcgttctgcaccaggggtaagatggcctccagcaccttgctggctgaccctggaagcatctccagtaccttcttatcaattgccattttgtccacaatggtcttaaagtagcgcagggcactgacaacttccttctctttctcctccagccagctcaggttcttctgcctttgagacctggaagccacagcactggtggacataaattctactgcctgctgctccagatccaaggggagagggtagccctctggtagaaatctgtctgttgcctcctggaagagaggaaacctggattctttgttcacaggcttctctggaatctttacggacacctcagctggttttcccttctttgatggcgttctcttgattttgggtgagtggaatttgtccatcagcttcatggtgaaggaagagagatgagaacgctgagagtctggaacgacacctcctgtcctcttgttctgttccaaggttgtcaggctgggacgaaatcccaagaaagaaatgggcatgtggtcactatcatagcagactgccagttagggacatcagaatatatttctctgtcctcaagttaggaagtgagaggacaaacctggccttctgtgttgtttcagccactaattggttttgtcaattaggcaaaacataatttctctaagcctcttttctcatccacaggcattag

SEQ ID NO: 16451 - RNA, 4797 nt, Homo sapiens
  source 1..4797: mol_type = other RNA
gtcctaggaggctcctctgtggccaggcttctgcctccctgcaccctgagggaccattcgggtgcctcagggatgcccttccctcccaggggcactgacagcactggctgaaaggtctgaagagccagaggaggagccctgctggctggcccaggatggggcaaggagggagggaaagccaggggatggggagggacatgagatggagtttaaggcacacagcgagcgatggaggagggaggtgctggcctctcccctctgaattaactcccccaggagctcagctctggcctcagtttggtgaggttcagaagactcccagcaataaaaagtatttcttggatgatcaagtcctcccttactccagcctcctcttctcagctccccaggtggtgtgggaggggcccagtggcctggggtggggggtaaggggcgacgggatgacagagactgctgctgctctcaggcgggcaagggaggccctgatggcgccagtaccgcggggcagagcaccagctgcggggctgctaaggcgtcacctgcgtacctttccgggcctgctgaaaagctcacaccatcctccatgcatcagaaggggaagcggaaagtgaaaggatcctcccccgagtctactctgcattctgcccacccagctgcttgcccccattccagggcccctgcaggacaggccaccccaggaggcctccactcatttgagatttcagaagattcagggaccctggagcttagggagggggagcacccaccacttccttggtctgctgatgaggtctctgctgctctctccctggaggggagtgggtggaaggtcaagaggggagagatggaagtaaaagcagaaaacaaaaccaaaccagaaaaccaccggtttgtaaattggcaacaagacctgcctgctggctgccctgaggcccacgggtctgctcccacagaggaaggaggcaggaagcggctggcaggctccagctcccgcccggccccgctgagggctggccagcctcatggctccgaggccgggactcctgccatgcgcctaacaggtccaaggtcctctccggtctgggagctgccctctgcgcccctcgagcattctcctggatcccggcgtctgctcctaggtcttctcttcccggtctgtttttctccttgttatgttcctgggtttaattttcagagacagttcccatagggcctcctcagccaggtggtcactgaagtcattgaagaagtttataatgtcgtcgttcctccgcatgtcatagtgcgcctgctggaagcagcgcatgctgtcgaggatgttgaactgctgccaccgcttggagaagttcactttcccgtcgatgtagtctgggtttcccaggtgaacgaaggtcaggtcctgcaggatcagccccaggtacgggatgcacggcggttccacctccgagagggcggcccggtaggctcggaaggaggacgagctgtcgatcagtgtgcagtactcggccaggccctctgaagtctgcttctgccactccagcctgcggatgggcgccgagtccagggcagagaggatggccaagtaggagttgaagttattcagcttccgcaagtgcttcatgatcttgatgaacttcaagagcagccgttccctgtcctgggccttttcctgtaacatgattatggaccggacccagtaggacatgttgttgaagtgctccgtgaactgggtcaagttggggctcttctcctcattctgctcttttgcccaaagcaaaacctcaggaatctctattttatagaagagctcagcatccagcagcgttagctgctccgctatctcatggctgtgaaagtcgtgcaaggtccccggcctggctgctaccccccgggctgccaggggctggctggaggtggcacacctgagtagcttcttctggtccaccttgtccaggatgttcttccggagcacacgggccaggctcagctccccattgcacaccaggcggaagaccagttccatcagcagcttcaggatctcttctgtcaactccaccaggcagagctcatccaccacccgtaccagcacgaagaacgtgttcttgctgacgcgcttcttgaatgtgtcggcaaagggagagaatttctcatatctgtactgcagcttcttgatgagctcctctggggagatgaaggtcctgtaggtggtcaggaatgcctcgcagtacaacaccaaatctttcctgtcagtctcagtagcatggaccagtaagatgtccccagatcctccgcggacgtccggcccgtcatcaccctcctgcttgagcgtcagcctggacataatttcgttgtggtcaatgagggacagctcgtccacttcctcctccgactgagccgactccagagcatctggtgactttggggccctctcactgccgtctctgctgtccttcccagggacgccgctgaccgctgagggatctctgggatgtccgtctttcccagccggtggctccgagggcacgggcaagctgccgtgccggctgagaaaggagttagagacggacacactgaggccctgagcggcactgccgtcctcgggggtgaaggccactttagtttgctggacacagtgggagacagaggagaaggaagaagcagcacaggaggcctgcagctgccgctgcttggggggtagggcgggcggcggggccagctcctgcacggagtccaccccactgaaggagtcgctgaagccgtatacctccatgaggagcttgttcttctgctggtagatgtgctcgttctgtggcgtctggtagaacatagagggctgcggctccgagtagtcctccagcaactgcatgtaggccagcatgtgtttgtttttcttctctggtagaggaggtggtttttctgggtcaccggttgactcaggagcagtaaaatcacccacaaattcgacaggggctgaggaacctccatgctgaaagggcagaatagcagcaaagggcgcgtaggggacggatgggatcggggctgtgctctgcaggtcctccccagagatgttgtcatactgcgagggatgccgctcgtaggacaccctgcagccagagccgtccgccgtctgggaggctgcgctcctgcgcttcttctcggggagagcaggtggcgtatctgtctgctgccctggggccagaggtccgtctggctggggatggccgccaagaggcagctggaaaggagggccaagaaatggagacccagactcccccaaagactctggcaacgggctaaggttccaggccgtctgctgaggtatctggtctgcgttagagaggtcttgctggaggaattcatagtcgggatcatagtggtctagtgtttcacagcttgtgttccgggagcactgcccactgtccctgtccagagaggacagctgctcgtctgacttgctgagcttgcctatgctgctgcagggggagaggcggggcgactctccaccatatgagtggctgcctcctgacagtcgcctctgtgcgtaacagtcaacatcaaaatcctgcctattgattccaacaggcaaactggagccactggtggctcggctcatgggggccaccacagccactcgggtaggggacggcgccgactgtcttttcttgggtggcaatgctggtggaggactattatcaaccacccgaatgccaggcagaggaggcttggggggcgcgacctcttcatccgtggcatctgggaggagctcagttgactgtgacatcccagtcgtcttgtttaggatctctacctcgcggtctgtcagggggagctctgctgggccatcaggcttgctggcaggggaactgggcttcacggggctcgtcggagacggacgtccctgcttctcgatggtgagcctgaccagctccttcactccatccagcacagccttgatgacccccttcacagtcgtcaccatctccttgtcttctgagttcacgccttccagcatcacttggtcagaccagcgaatgaggttggcgaggctttggtacactcggctatagcaggaagagagggctgagctgtgctgaattcgaggatcgttctgcaccaggggtaagatggcctccagcaccttgctggctgaccctggaagcatctccagtaccttcttatcaattgccattttgtccacaatggtcttaaagtagcgcagggcactgacaacttccttctctttctcctccagccagctcaggttcttctgcctttgagacctggaagccacagcactggtggacataaattctactgcctgctgctccagatccaaggggagagggtagccctctggtagaaatctgtctgttgcctcctggaagagaggaaacctggattctttgttcacaggcttctctggaatctttacggacacctcagctggttttcccttctttgatggcgttctcttgattttgggtgagtggaatttgtccatcagcttcatggtgaaggaagagagatgagaacgctgagagtctggaacgacacctcctgtcctcttgttctgttccaaggttgtcaggctgggacgaaatcccaagaaagaaatgggcatgtggtcactatcatagcagactgccagttagggacatcagaatatatttctctgtcctcaagttaggaagtgagaggacaaacctggccttctgtgttgtttcagccactaattggttttgtcaattaggcaaaacataatttctctaagcctcttttctcatccacaggcattag

SEQ ID NO: 16452 - RNA, 4896 nt, Homo sapiens
  source 1..4896: mol_type = other RNA
gtcctaggaggctcctctgtggccaggcttctgcctccctgcaccctgagggaccattcgggtgcctcagggatgcccttccctcccaggggcactgacagcactggctgaaaggtctgaagagccagaggaggagccctgctggctggcccaggatggggcaaggagggagggaaagccaggggatggggagggacatgagatggagtttaaggcacacagcgagcgatggaggagggaggtgctggcctctcccctctgaattaactcccccaggagctcagctctggcctcagtttggtgaggttcagaagactcccagcaataaaaagtatttcttggatgatcaagtcctcccttactccagcctcctcttctcagctccccaggtggtgtgggaggggcccagtggcctggggtggggggtaaggggcgacgggatgacagagactgctgctgctctcaggcgggcaagggaggccctgatggcgccagtaccgcggggcagagcaccagctgcggggctgctaaggcgtcacctgcgtacctttccgggcctgctgaaaagctcacaccatcctccatgcatcagaaggggaagcggaaagtgaaaggatcctcccccgagtctactctgcattctgcccacccagctgcttgcccccattccagggcccctgcaggacaggccaccccaggaggcctccactcatttgagatttcagaagattcagggaccctggagcttagggagggggagcacccaccacttccttggtctgctgatgaggtctctgctgctctctccctggaggggagtgggtggaaggtcaagaggggagagatggaagtaaaagcagaaaacaaaaccaaaccagaaaaccaccggtttgtaaattggcaacaagacctgcctgctggctgccctgaggcccacgggtctgctcccacagaggaaggaggcaggaagcggctggcaggctccagctcccgcccggccccgctgagggctggccagcctcatggctccgaggccgggactcctgccatgcgcctaacaggtccaaggtcctctccggtctgggagctgccctctgcgcccctcgagcattctcctggatcccggcgtctgctcctaggtcttctcttcccggtctgtttttctccttgttatgttcctgggtttaattttcagagacagttcccatagggcctcctcagccaggtggtcactgaagtcattgaagaagtttataatgtcgtcgttcctccgcatgtcatagtgcgcctgctggaagcagcgcatgctgtcgaggatgttgaactgctgccaccgcttggagaagttcactttcccgtcgatgtagtctgggtttcccaggtgaacgaaggtcaggtcctgcaggatcagccccaggtacgggatgcacggcggttccacctccgagagggcggcccggtaggctcggaaggaggacgagctgtcgatcagtgtgcagtactcggccaggccctctgaagtctgcttctgccactccagcctgcggatgggcgccgagtccagggcagagaggatggccaagtaggagttgaagttattcagcttccgcaagtgcttcatgatcttgatgaacttcaagagcagccgttccctgtcctgggccttttcctgtaacatgattatggaccggacccagtaggacatgttgttgaagtgctccgtgaactgggtcaagttggggctcttctcctcattctgctcttttgcccaaagcaaaacctcaggaatctctattttatagaagagctcagcatccagcagcgttagctgctccgctatctcatggctgtgaaagtcgtgcaaggtccccggcctggctgctaccccccgggctgccaggggctggctggaggtggcacacctgagtagcttcttctggtccaccttgtccaggatgttcttccggagcacacgggccaggctcagctccccattgcacaccaggcggaagaccagttccatcagcagcttcaggatctcttctgtcaactccaccaggcagagctcatccaccacccgtaccagcacgaagaacgtgttcttgctgacgcgcttcttgaatgtgtcggcaaagggagagaatttctcatatctgtactgcagcttcttgatgagctcctctggggagatgaaggtcctgtaggtggtcaggaatgcctcgcagtacaacaccaaatctttcctgtcagtctcagtagcatggaccagtaagatgtccccagatcctccgcggacgtccggcccgtcatcaccctcctgcttgagcgtcagcctggacataatttcgttgtggtcaatgagggacagctcgtccacttcctcctccgactgagccgactccagagcatctggtgactttggggccctctcactgccgtctctgctgtccttcccagggacgccgctgaccgctgagggatctctgggatgtccgtctttcccagccggtggctccgagtcagtgaaagaggtttcggaaggaaggcagacagtattcccatgaaagctgctctcctgagaagccgagagaggcccgtccacggtgctgggaggtggaccggccatggttggcacggctaagtcagagctctgagactggtgggcaggtgggaaatgtggagaggaagaggaggtaggcggaaggaaaggcggaacggaagcttggtggtgaggcacgaaatcctgggagtaggacctaaacacagacttatacagctgccgctgcttggggggtagggcgggcggcggggccagctcctgcacggagtccaccccactgaaggagtcgctgaagccgtatacctccatgaggagcttgttcttctgctggtagatgtgctcgttctgtggcgtctggtagaacatagagggctgcggctccgagtagtcctccagcaactgcatgtaggccagcatgtgtttgtttttcttctctggtagaggaggtggtttttctgggtcaccggttgactcaggagcagtaaaatcacccacaaattcgacaggggctgaggaacctccatgctgaaagggcagaatagcagcaaagggcgcgtaggggacggatgggatcggggctgtgctctgcaggtcctccccagagatgttgtcatactgcgagggatgccgctcgtaggacaccctgcagccagagccgtccgccgtctgggaggctgcgctcctgcgcttcttctcggggagagcaggtggcgtatctgtctgctgccctggggccagaggtccgtctggctggggatggccgccaagaggcagctggaaaggagggccaagaaatggagacccagactcccccaaagactctggcaacgggctaaggttccaggccgtctgctgaggtatctggtctgcgttagagaggtcttgctggaggaattcatagtcgggatcatagtggtctagtgtttcacagcttgtgttccgggagcactgcccactgtccctgtccagagaggacagctgctcgtctgacttgctgagcttgcctatgctgctgcagggggagaggcggggcgactctccaccatatgagtggctgcctcctgacagtcgcctctgtgcgtaacagtcaacatcaaaatcctgcctattgattccaacaggcaaactggagccactggtggctcggctcatgggggccaccacagccactcgggtaggggacggcgccgactgtcttttcttgggtggcaatgctggtggaggactattatcaaccacccgaatgccaggcagaggaggcttggggggcgcgacctcttcatccgtggcatctgggaggagctcagttgactgtgacatcccagtcgtcttgtttaggatctctacctcgcggtctgtcagggggagctctgctgggccatcaggcttgctggcaggggaactgggcttcacggggctcgtcggagacggacgtccctgcttctcgatggtgagcctgaccagctccttcactccatccagcacagccttgatgacccccttcacagtcgtcaccatctccttgtcttctgagttcacgccttccagcatcacttggtcagaccagcgaatgaggttggcgaggctttggtacactcggctatagcaggaagagagggctgagctgtgctgaattcgaggatcgttctgcaccaggggtaagatggcctccagcaccttgctggctgaccctggaagcatctccagtaccttcttatcaattgccattttgtccacaatggtcttaaagtagcgcagggcactgacaacttccttctctttctcctccagccagctcaggttcttctgcctttgagacctggaagccacagcactggtggacataaattctactgcctgctgctccagatccaaggggagagggtagccctctggtagaaatctgtctgttgcctcctggaagagaggaaacctggattctttgttcacaggcttctctggaatctttacggacacctcagctggttttcccttctttgatggcgttctcttgattttgggtgagtggaatttgtccatcagcttcatggtgaaggaagagagatgagaacgctgagagtctggaacgacacctcctgtcctcttgttctgttccaaggttgtcaggctgggacgaaatcccaagaaagaaatgggcatgtggtcactatcatagcagactgccagttagggacatcagaatatatttctctgtcctcaagttaggaagtgagaggacaaacctggccttctgtgttgtttcagccactaattggttttgtcaattaggcaaaacataatttctctaagcctcttttctcatccacaggcattag

SEQ ID NO: 16453 - RNA, 5052 nt, Homo sapiens
  source 1..5052: mol_type = other RNA
gtcctaggaggctcctctgtggccaggcttctgcctccctgcaccctgagggaccattcgggtgcctcagggatgcccttccctcccaggggcactgacagcactggctgaaaggtctgaagagccagaggaggagccctgctggctggcccaggatggggcaaggagggagggaaagccaggggatggggagggacatgagatggagtttaaggcacacagcgagcgatggaggagggaggtgctggcctctcccctctgaattaactcccccaggagctcagctctggcctcagtttggtgaggttcagaagactcccagcaataaaaagtatttcttggatgatcaagtcctcccttactccagcctcctcttctcagctccccaggtggtgtgggaggggcccagtggcctggggtggggggtaaggggcgacgggatgacagagactgctgctgctctcaggcgggcaagggaggccctgatggcgccagtaccgcggggcagagcaccagctgcggggctgctaaggcgtcacctgcgtacctttccgggcctgctgaaaagctcacaccatcctccatgcatcagaaggggaagcggaaagtgaaaggatcctcccccgagtctactctgcattctgcccacccagctgcttgcccccattccagggcccctgcaggacaggccaccccaggaggcctccactcatttgagatttcagaagattcagggaccctggagcttagggagggggagcacccaccacttccttggtctgctgatgaggtctctgctgctctctccctggaggggagtgggtggaaggtcaagaggggagagatggaagtaaaagcagaaaacaaaaccaaaccagaaaaccaccggtttgtaaattggcaacaagacctgcctgctggctgccctgaggcccacgggtctgctcccacagaggaaggaggcaggaagcggctggcaggctccagctcccgcccggccccgctgagggctggccagcctcatggctccgaggccgggactcctgccatgcgcctaacaggtccaaggtcctctccggtctgggagctgccctctgcgcccctcgagcattctcctggatcccggcgtctgctcctaggtcttctcttcccggtctgtttttctccttgttatgttcctgggtttaattttcagagacagttcccatagggcctcctcagccaggtggtcactgaagtcattgaagaagtttataatgtcgtcgttcctccgcatgtcatagtgcgcctgctggaagcagcgcatgctgtcgaggatgttgaactgctgccaccgcttggagaagttcactttcccgtcgatgtagtctgggtttcccaggtgaacgaaggtcaggtcctgcaggatcagccccaggtacgggatgcacggcggttccacctccgagagggcggcccggtaggctcggaaggaggacgagctgtcgatcagtgtgcagtactcggccaggccctctgaagtctgcttctgccactccagcctgcggatgggcgccgagtccagggcagagaggatggccaagtaggagttgaagttattcagcttccgcaagtgcttcatgatcttgatgaacttcaagagcagccgttccctgtcctgggccttttcctgtaacatgattatggaccggacccagtaggacatgttgttgaagtgctccgtgaactgggtcaagttggggctcttctcctcattctgctcttttgcccaaagcaaaacctcaggaatctctattttatagaagagctcagcatccagcagcgttagctgctccgctatctcatggctgtgaaagtcgtgcaaggtccccggcctggctgctaccccccgggctgccaggggctggctggaggtggcacacctgagtagcttcttctggtccaccttgtccaggatgttcttccggagcacacgggccaggctcagctccccattgcacaccaggcggaagaccagttccatcagcagcttcaggatctcttctgtcaactccaccaggcagagctcatccaccacccgtaccagcacgaagaacgtgttcttgctgacgcgcttcttgaatgtgtcggcaaagggagagaatttctcatatctgtactgcagcttcttgatgagctcctctggggagatgaaggtcctgtaggtggtcaggaatgcctcgcagtacaacaccaaatctttcctgtcagtctcagtagcatggaccagtaagatgtccccagatcctccgcggacgtccggcccgtcatcaccctcctgcttgagcgtcagcctggacataatttcgttgtggtcaatgagggacagctcgtccacttcctcctccgactgagccgactccagagcatctggtgactttggggccctctcactgccgtctctgctgtccttcccagggacgccgctgaccgctgagggatctctgggatgtccgtctttcccagccggtggctccgagtcagtgaaagaggtttcggaaggaaggcagacagtattcccatgaaagctgctctcctgagaagccgagagaggcccgtccacggtgctgggaggtggaccggccatggttggcacggctaagtcagagctctgagactggtgggcaggtgggaaatgtggagaggaagaggaggtaggcggaaggaaaggcggaacggaagcttggtggtgaggcacgaaatcctgggagtaggacctaaacacagacttatacgagggcacgggcaagctgccgtgccggctgagaaaggagttagagacggacacactgaggccctgagcggcactgccgtcctcgggggtgaaggccactttagtttgctggacacagtgggagacagaggagaaggaagaagcagcacaggaggccagctgccgctgcttggggggtagggcgggcggcggggccagctcctgcacggagtccaccccactgaaggagtcgctgaagccgtatacctccatgaggagcttgttcttctgctggtagatgtgctcgttctgtggcgtctggtagaacatagagggctgcggctccgagtagtcctccagcaactgcatgtaggccagcatgtgtttgtttttcttctctggtagaggaggtggtttttctgggtcaccggttgactcaggagcagtaaaatcacccacaaattcgacaggggctgaggaacctccatgctgaaagggcagaatagcagcaaagggcgcgtaggggacggatgggatcggggctgtgctctgcaggtcctccccagagatgttgtcatactgcgagggatgccgctcgtaggacaccctgcagccagagccgtccgccgtctgggaggctgcgctcctgcgcttcttctcggggagagcaggtggcgtatctgtctgctgccctggggccagaggtccgtctggctggggatggccgccaagaggcagctggaaaggagggccaagaaatggagacccagactcccccaaagactctggcaacgggctaaggttccaggccgtctgctgaggtatctggtctgcgttagagaggtcttgctggaggaattcatagtcgggatcatagtggtctagtgtttcacagcttgtgttccgggagcactgcccactgtccctgtccagagaggacagctgctcgtctgacttgctgagcttgcctatgctgctgcagggggagaggcggggcgactctccaccatatgagtggctgcctcctgacagtcgcctctgtgcgtaacagtcaacatcaaaatcctgcctattgattccaacaggcaaactggagccactggtggctcggctcatgggggccaccacagccactcgggtaggggacggcgccgactgtcttttcttgggtggcaatgctggtggaggactattatcaaccacccgaatgccaggcagaggaggcttggggggcgcgacctcttcatccgtggcatctgggaggagctcagttgactgtgacatcccagtcgtcttgtttaggatctctacctcgcggtctgtcagggggagctctgctgggccatcaggcttgctggcaggggaactgggcttcacggggctcgtcggagacggacgtccctgcttctcgatggtgagcctgaccagctccttcactccatccagcacagccttgatgacccccttcacagtcgtcaccatctccttgtcttctgagttcacgccttccagcatcacttggtcagaccagcgaatgaggttggcgaggctttggtacactcggctatagcaggaagagagggctgagctgtgctgaattcgaggatcgttctgcaccaggggtaagatggcctccagcaccttgctggctgaccctggaagcatctccagtaccttcttatcaattgccattttgtccacaatggtcttaaagtagcgcagggcactgacaacttccttctctttctcctccagccagctcaggttcttctgcctttgagacctggaagccacagcactggtggacataaattctactgcctgctgctccagatccaaggggagagggtagccctctggtagaaatctgtctgttgcctcctggaagagaggaaacctggattctttgttcacaggcttctctggaatctttacggacacctcagctggttttcccttctttgatggcgttctcttgattttgggtgagtggaatttgtccatcagcttcatggtgaaggaagagagatgagaacgctgagagtctggaacgacacctcctgtcctcttgttctgttccaaggttgtcaggctgggacgaaatcccaagaaagaaatgggcatgtggtcactatcatagcagactgccagttagggacatcagaatatatttctctgtcctcaagttaggaagtgagaggacaaacctggccttctgtgttgtttcagccactaattggttttgtcaattaggcaaaacataatttctctaagcctcttttctcatccacaggcattag

SEQ ID NO: 16454 - RNA, 5055 nt, Homo sapiens
  source 1..5055: mol_type = other RNA
gtcctaggaggctcctctgtggccaggcttctgcctccctgcaccctgagggaccattcgggtgcctcagggatgcccttccctcccaggggcactgacagcactggctgaaaggtctgaagagccagaggaggagccctgctggctggcccaggatggggcaaggagggagggaaagccaggggatggggagggacatgagatggagtttaaggcacacagcgagcgatggaggagggaggtgctggcctctcccctctgaattaactcccccaggagctcagctctggcctcagtttggtgaggttcagaagactcccagcaataaaaagtatttcttggatgatcaagtcctcccttactccagcctcctcttctcagctccccaggtggtgtgggaggggcccagtggcctggggtggggggtaaggggcgacgggatgacagagactgctgctgctctcaggcgggcaagggaggccctgatggcgccagtaccgcggggcagagcaccagctgcggggctgctaaggcgtcacctgcgtacctttccgggcctgctgaaaagctcacaccatcctccatgcatcagaaggggaagcggaaagtgaaaggatcctcccccgagtctactctgcattctgcccacccagctgcttgcccccattccagggcccctgcaggacaggccaccccaggaggcctccactcatttgagatttcagaagattcagggaccctggagcttagggagggggagcacccaccacttccttggtctgctgatgaggtctctgctgctctctccctggaggggagtgggtggaaggtcaagaggggagagatggaagtaaaagcagaaaacaaaaccaaaccagaaaaccaccggtttgtaaattggcaacaagacctgcctgctggctgccctgaggcccacgggtctgctcccacagaggaaggaggcaggaagcggctggcaggctccagctcccgcccggccccgctgagggctggccagcctcatggctccgaggccgggactcctgccatgcgcctaacaggtccaaggtcctctccggtctgggagctgccctctgcgcccctcgagcattctcctggatcccggcgtctgctcctaggtcttctcttcccggtctgtttttctccttgttatgttcctgggtttaattttcagagacagttcccatagggcctcctcagccaggtggtcactgaagtcattgaagaagtttataatgtcgtcgttcctccgcatgtcatagtgcgcctgctggaagcagcgcatgctgtcgaggatgttgaactgctgccaccgcttggagaagttcactttcccgtcgatgtagtctgggtttcccaggtgaacgaaggtcaggtcctgcaggatcagccccaggtacgggatgcacggcggttccacctccgagagggcggcccggtaggctcggaaggaggacgagctgtcgatcagtgtgcagtactcggccaggccctctgaagtctgcttctgccactccagcctgcggatgggcgccgagtccagggcagagaggatggccaagtaggagttgaagttattcagcttccgcaagtgcttcatgatcttgatgaacttcaagagcagccgttccctgtcctgggccttttcctgtaacatgattatggaccggacccagtaggacatgttgttgaagtgctccgtgaactgggtcaagttggggctcttctcctcattctgctcttttgcccaaagcaaaacctcaggaatctctattttatagaagagctcagcatccagcagcgttagctgctccgctatctcatggctgtgaaagtcgtgcaaggtccccggcctggctgctaccccccgggctgccaggggctggctggaggtggcacacctgagtagcttcttctggtccaccttgtccaggatgttcttccggagcacacgggccaggctcagctccccattgcacaccaggcggaagaccagttccatcagcagcttcaggatctcttctgtcaactccaccaggcagagctcatccaccacccgtaccagcacgaagaacgtgttcttgctgacgcgcttcttgaatgtgtcggcaaagggagagaatttctcatatctgtactgcagcttcttgatgagctcctctggggagatgaaggtcctgtaggtggtcaggaatgcctcgcagtacaacaccaaatctttcctgtcagtctcagtagcatggaccagtaagatgtccccagatcctccgcggacgtccggcccgtcatcaccctcctgcttgagcgtcagcctggacataatttcgttgtggtcaatgagggacagctcgtccacttcctcctccgactgagccgactccagagcatctggtgactttggggccctctcactgccgtctctgctgtccttcccagggacgccgctgaccgctgagggatctctgggatgtccgtctttcccagccggtggctccgagtcagtgaaagaggtttcggaaggaaggcagacagtattcccatgaaagctgctctcctgagaagccgagagaggcccgtccacggtgctgggaggtggaccggccatggttggcacggctaagtcagagctctgagactggtgggcaggtgggaaatgtggagaggaagaggaggtaggcggaaggaaaggcggaacggaagcttggtggtgaggcacgaaatcctgggagtaggacctaaacacagacttatacgagggcacgggcaagctgccgtgccggctgagaaaggagttagagacggacacactgaggccctgagcggcactgccgtcctcgggggtgaaggccactttagtttgctggacacagtgggagacagaggagaaggaagaagcagcacaggaggcctgcagctgccgctgcttggggggtagggcgggcggcggggccagctcctgcacggagtccaccccactgaaggagtcgctgaagccgtatacctccatgaggagcttgttcttctgctggtagatgtgctcgttctgtggcgtctggtagaacatagagggctgcggctccgagtagtcctccagcaactgcatgtaggccagcatgtgtttgtttttcttctctggtagaggaggtggtttttctgggtcaccggttgactcaggagcagtaaaatcacccacaaattcgacaggggctgaggaacctccatgctgaaagggcagaatagcagcaaagggcgcgtaggggacggatgggatcggggctgtgctctgcaggtcctccccagagatgttgtcatactgcgagggatgccgctcgtaggacaccctgcagccagagccgtccgccgtctgggaggctgcgctcctgcgcttcttctcggggagagcaggtggcgtatctgtctgctgccctggggccagaggtccgtctggctggggatggccgccaagaggcagctggaaaggagggccaagaaatggagacccagactcccccaaagactctggcaacgggctaaggttccaggccgtctgctgaggtatctggtctgcgttagagaggtcttgctggaggaattcatagtcgggatcatagtggtctagtgtttcacagcttgtgttccgggagcactgcccactgtccctgtccagagaggacagctgctcgtctgacttgctgagcttgcctatgctgctgcagggggagaggcggggcgactctccaccatatgagtggctgcctcctgacagtcgcctctgtgcgtaacagtcaacatcaaaatcctgcctattgattccaacaggcaaactggagccactggtggctcggctcatgggggccaccacagccactcgggtaggggacggcgccgactgtcttttcttgggtggcaatgctggtggaggactattatcaaccacccgaatgccaggcagaggaggcttggggggcgcgacctcttcatccgtggcatctgggaggagctcagttgactgtgacatcccagtcgtcttgtttaggatctctacctcgcggtctgtcagggggagctctgctgggccatcaggcttgctggcaggggaactgggcttcacggggctcgtcggagacggacgtccctgcttctcgatggtgagcctgaccagctccttcactccatccagcacagccttgatgacccccttcacagtcgtcaccatctccttgtcttctgagttcacgccttccagcatcacttggtcagaccagcgaatgaggttggcgaggctttggtacactcggctatagcaggaagagagggctgagctgtgctgaattcgaggatcgttctgcaccaggggtaagatggcctccagcaccttgctggctgaccctggaagcatctccagtaccttcttatcaattgccattttgtccacaatggtcttaaagtagcgcagggcactgacaacttccttctctttctcctccagccagctcaggttcttctgcctttgagacctggaagccacagcactggtggacataaattctactgcctgctgctccagatccaaggggagagggtagccctctggtagaaatctgtctgttgcctcctggaagagaggaaacctggattctttgttcacaggcttctctggaatctttacggacacctcagctggttttcccttctttgatggcgttctcttgattttgggtgagtggaatttgtccatcagcttcatggtgaaggaagagagatgagaacgctgagagtctggaacgacacctcctgtcctcttgttctgttccaaggttgtcaggctgggacgaaatcccaagaaagaaatgggcatgtggtcactatcatagcagactgccagttagggacatcagaatatatttctctgtcctcaagttaggaagtgagaggacaaacctggccttctgtgttgtttcagccactaattggttttgtcaattaggcaaaacataatttctctaagcctcttttctcatccacaggcattag

SEQ ID NO: 16455 - RNA, 4731 nt, Homo sapiens
  source 1..4731: mol_type = other RNA
gtcctaggaggctcctctgtggccaggcttctgcctccctgcaccctgagggaccattcgggtgcctcagggatgcccttccctcccaggggcactgacagcactggctgaaaggtctgaagagccagaggaggagccctgctggctggcccaggatggggcaaggagggagggaaagccaggggatggggagggacatgagatggagtttaaggcacacagcgagcgatggaggagggaggtgctggcctctcccctctgaattaactcccccaggagctcagctctggcctcagtttggtgaggttcagaagactcccagcaataaaaagtatttcttggatgatcaagtcctcccttactccagcctcctcttctcagctccccaggtggtgtgggaggggcccagtggcctggggtggggggtaaggggcgacgggatgacagagactgctgctgctctcaggcgggcaagggaggccctgatggcgccagtaccgcggggcagagcaccagctgcggggctgctaaggcgtcacctgcgtacctttccgggcctgctgaaaagctcacaccatcctccatgcatcagaaggggaagcggaaagtgaaaggatcctcccccgagtctactctgcattctgcccacccagctgcttgcccccattccagggcccctgcaggacaggccaccccaggaggcctccactcatttgagatttcagaagattcagggaccctggagcttagggagggggagcacccaccacttccttggtctgctgatgaggtctctgctgctctctccctggaggggagtgggtggaaggtcaagaggggagagatggaagtaaaagcagaaaacaaaaccaaaccagaaaaccaccggtttgtaaattggcaacaagacctgcctgctggctgccctgaggcccacgggtctgctcccacagaggaaggaggcaggaagcggctggcaggctccagctcccgcccggccccgctgagggctggccagcctcatggctccgaggccgggactcctgccatgcgcctaacaggtccaaggtcctctccggtctgggagctgccctctgcgcccctcgagcattctcctggatcccggcgtctgctcctaggtcttctcttcccggtctgtttttctccttgttatgttcctgggtttaattttcagagacagttcccatagggcctcctcagccaggtggtcactgaagtcattgaagaagtttataatgtcgtcgttcctccgcatgtcatagtgcgcctgctggaagcagcgcatgctgtcgaggatgttgaactgctgccaccgcttggagaagttcactttcccgtcgatgtagtctgggtttcccaggtgaacgaaggtcaggtcctgcaggatcagccccaggtacgggatgcacggcggttccacctccgagagggcggcccggtaggctcggaaggaggacgagctgtcgatcagtgtgcagtactcggccaggccctctgaagtctgcttctgccactccagcctgcggatgggcgccgagtccagggcagagaggatggccaagtaggagttgaagttattcagcttccgcaagtgcttcatgatcttgatgaacttcaagagcagccgttccctgtcctgggccttttcctgtaacatgattatggaccggacccagtaggacatgttgttgaagtgctccgtgaactgggtcaagttggggctcttctcctcattctgctcttttgcccaaagcaaaacctcaggaatctctattttatagaagagctcagcatccagcagcgttagctgctccgctatctcatggctgtgaaagtcgtgcaaggtccccggcctggctgctaccccccgggctgccaggggctggctggaggtggcacacctgagtagcttcttctggtccaccttgtccaggatgttcttccggagcacacgggccaggctcagctccccattgcacaccaggcggaagaccagttccatcagcagcttcaggatctcttctgtcaactccaccaggcagagctcatccaccacccgtaccagcacgaagaacgtgttcttgctgacgcgcttcttgaatgtgtcggcaaagggagagaatttctcatatctgtactgcagcttcttgatgagctcctctggggagatgaaggtcctgtaggtggtcaggaatgcctcgcagtacaacaccaaatctttcctgtcagtctcagtagcatggaccagtaagatgtccccagatcctccgcggacgtccggcccgtcatcaccctcctgcttgagcgtcagcctggacataatttcgttgtggtcaatgagggacagctcgtccacttcctcctccgactgagccgactccagagcatctggtgactttggggccctctcactgccgtctctgctgtccttcccagggacgccgctgaccgctgagggatctctgggatgtccgtctttcccagccggtggctctcctcgagagggagccagctcctcgctgctctggccagaggaatacagattgacatattcaccctcaccagcttcctcactggcgttttcactcagctgccgctgcttggggggtagggcgggcggcggggccagctcctgcacggagtccaccccactgaaggagtcgctgaagccgtatacctccatgaggagcttgttcttctgctggtagatgtgctcgttctgtggcgtctggtagaacatagagggctgcggctccgagtagtcctccagcaactgcatgtaggccagcatgtgtttgtttttcttctctggtagaggaggtggtttttctgggtcaccggttgactcaggagcagtaaaatcacccacaaattcgacaggggctgaggaacctccatgctgaaagggcagaatagcagcaaagggcgcgtaggggacggatgggatcggggctgtgctctgcaggtcctccccagagatgttgtcatactgcgagggatgccgctcgtaggacaccctgcagccagagccgtccgccgtctgggaggctgcgctcctgcgcttcttctcggggagagcaggtggcgtatctgtctgctgccctggggccagaggtccgtctggctggggatggccgccaagaggcagctggaaaggagggccaagaaatggagacccagactcccccaaagactctggcaacgggctaaggttccaggccgtctgctgaggtatctggtctgcgttagagaggtcttgctggaggaattcatagtcgggatcatagtggtctagtgtttcacagcttgtgttccgggagcactgcccactgtccctgtccagagaggacagctgctcgtctgacttgctgagcttgcctatgctgctgcagggggagaggcggggcgactctccaccatatgagtggctgcctcctgacagtcgcctctgtgcgtaacagtcaacatcaaaatcctgcctattgattccaacaggcaaactggagccactggtggctcggctcatgggggccaccacagccactcgggtaggggacggcgccgactgtcttttcttgggtggcaatgctggtggaggactattatcaaccacccgaatgccaggcagaggaggcttggggggcgcgacctcttcatccgtggcatctgggaggagctcagttgactgtgacatcccagtcgtcttgtttaggatctctacctcgcggtctgtcagggggagctctgctgggccatcaggcttgctggcaggggaactgggcttcacggggctcgtcggagacggacgtccctgcttctcgatggtgagcctgaccagctccttcactccatccagcacagccttgatgacccccttcacagtcgtcaccatctccttgtcttctgagttcacgccttccagcatcacttggtcagaccagcgaatgaggttggcgaggctttggtacactcggctatagcaggaagagagggctgagctgtgctgaattcgaggatcgttctgcaccaggggtaagatggcctccagcaccttgctggctgaccctggaagcatctccagtaccttcttatcaattgccattttgtccacaatggtcttaaagtagcgcagggcactgacaacttccttctctttctcctccagccagctcaggttcttctgcctttgagacctggaagccacagcactggtggacataaattctactgcctgctgctccagatccaaggggagagggtagccctctggtagaaatctgtctgttgcctcctggaagagaggaaacctggattctttgttcacaggcttctctggaatctttacggacacctcagctggttttcccttctttgatggcgttctcttgattttgggtgagtggaatttgtccatcagcttcatggtgaaggaagagagatgagaacgctgagagtctggaacgacacctcctgtcctcttgttctgttccaaggttgtcaggctgggacgaaatcccaagaaagaaatgggcatgtggtcactatcatagcagactgccagttagggacatcagaatatatttctctgtcctcaagttaggaagtgagaggacaaacctggccttctgtgttgtttcagccactaattggttttgtcaattaggcaaaacataatttctctaagcctcttttctcatccacaggcattag

SEQ ID NO: 16456 - RNA, 4526 nt, Homo sapiens
  source 1..4526: mol_type = other RNA
gtcctaggaggctcctctgtggccaggcttctgcctccctgcaccctgagggaccattcgggtgcctcagggatgcccttccctcccaggggcactgacagcactggctgaaaggtctgaagagccagaggaggagccctgctggctggcccaggatggggcaaggagggagggaaagccaggggatggggagggacatgagatggagtttaaggcacacagcgagcgatggaggagggaggtgctggcctctcccctctgaattaactcccccaggagctcagctctggcctcagtttggtgaggttcagaagactcccagcaataaaaagtatttcttggatgatcaagtcctcccttactccagcctcctcttctcagctccccaggtggtgtgggaggggcccagtggcctggggtggggggtaaggggcgacgggatgacagagactgctgctgctctcaggcgggcaagggaggccctgatggcgccagtaccgcggggcagagcaccagctgcggggctgctaaggcgtcacctgcgtacctttccgggcctgctgaaaagctcacaccatcctccatgcatcagaaggggaagcggaaagtgaaaggatcctcccccgagtctactctgcattctgcccacccagctgcttgcccccattccagggcccctgcaggacaggccaccccaggaggcctccactcatttgagatttcagaagattcagggaccctggagcttagggagggggagcacccaccacttccttggtctgctgatgaggtctctgctgctctctccctggaggggagtgggtggaaggtcaagaggggagagatggaagtaaaagcagaaaacaaaaccaaaccagaaaaccaccggtttgtaaattggcaacaagacctgcctgctggctgccctgaggcccacgggtctgctcccacagaggaaggaggcaggaagcggctggcaggctccagctcccgcccggccccgctgagggctggccagcctcatggctccgaggccgggactcctgccatgcgcctaacaggtccaaggtcctctccggtctgggagctgccctctgcgcccctcgagcattctcctggatcccggcgtctgctcctaggtcttctcttcccggtctgtttttctccttgttatgttcctgggtttaattttcagagacagttcccatagggcctcctcagccaggtggtcactgaagtcattgaagaagtttataatgtcgtcgttcctccgcatgtcatagtgcgcctgctggaagcagcgcatgctgtcgaggatgttgaactgctgccaccgcttggagaagttcactttcccgtcgatgtagtctgggtttcccaggtgaacgaaggtcaggtcctgcaggatcagccccaggtacgggatgcacggcggttccacctccgagagggcggcccggtaggctcggaaggaggacgagctgtcgatcagtgtgcagtactcggccaggccctctgaagtctgcttctgccactccagcctgcggatgggcgccgagtccagggcagagaggatggccaagtaggagttgaagttattcagcttccgcaagtgcttcatgatcttgatgaacttcaagagcagccgttccctgtcctgggccttttcctgtaacatgattatggaccggacccagtaggacatgttgttgaagtgctccgtgaactgggtcaagttggggctcttctcctcattctgctcttttgcccaaagcaaaacctcaggaatctctattttatagaagagctcagcatccagcagcgttagctgctccgctatctcatggctgtgaaagtcgtgcaaggtccccggcctggctgctaccccccgggctgccaggggctggctggaggtggcacacctgagtagcttcttctggtccaccttgtccaggatgttcttccggagcacacgggccaggctcagctccccattgcacaccaggcggaagaccagttccatcagcagcttcaggatctcttctgtcaactccaccaggcagagctcatccaccacccgtaccagcacgaagaacgtgttcttgctgacgcgcttcttgaatgtgtcggcaaagggagagaatttctcatatctgtactgcagcttcttgatgagctcctctggggagatgaaggtcctgtaggtggtcaggaatgcctcgcagtacaacaccaaatctttcctgtcagtctcagtagcatggaccagtaagatgtccccagatcctccgcggacgtccggcccgtcatcaccctcctgcttgagcgtcagcctggacataatttcgttgtggtcaatgagggacagctcgtccacttcctcctccgactgagccgactccagagcatctggtgactttggggccctctcactgccgtctctgctgtccttcccagggacgccgctgaccgctgagggatctctgggatgtccgtctttcccagccggtggctctcctcgagagggagccagctcctcgctgctctggccagaggaatacagattgacatattcaccctcaccagcttcctcactggcgttttcactcagctgccgctgcttggggggtagggcgggcggcggggccagctcctgcacggagtccaccccactgaaggagtcgctgaagccgtatacctccatgaggagcttgttcttctgctggtagatgtgctcgttctgtggcgtctggtagaacatagagggctgcggctccgagtagtcctccagcaactgcatgtaggccagcatgtgtttgtttttcttctctggtagaggaggtggtttttctgggtcaccggttgactcaggagcagtaaaatcacccacaaattcgacaggggctgaggaacctccatgctgaaagggcagaatagcagcaaagggcgcgtaggggacggatgggatcggggctgtgctctgcaggtcctccccagagatgttgtcatactgcgagggatgccgctcgtaggacaccctgcagccagagccgtccgccgtctgggaggctgcgctcctgcgcttcttctcggggagagcaggtggcgtatctgtctgctgccctggggccagaggtccgtctggctggggatggccgccaagaggcagctggaaaggagggccaagaaatggagacccagactcccccaaagactctggcaacgggctaaggttccaggccgtctgctgaggtatctggtctgcgttagagaggtcttgctggaggaattcatagtcgggatcatagtggtctagtgtttcacagcttgtgttccgggagcactgcccactgtccctgtccagagaggacagctgctcgtctgacttgctgagcttgcctatgctgctgcagggggagaggcggggcgactctccaccatatgagtggctgcctcctgacagtcgcctctgtgcgtaacagtcaacatcaaaatcctgcctattgattccaacaggcaaactggagccactggtggctcggctcatgggggccaccacagccactcgggtaggggacggcgccgactgtcttttcttgggtggcaatgctggtggaggactattatcaaccacccgaatgccaggcagaggaggcttggggggcgcgacctcttcatccgtggcatctgggaggagctcagttgactgtgacatcccagtcgtcttgtttaggatctctacctcgcggtctgtcagggggagctctgctgggccatcaggcttgctggcaggggaactgggcttcacggggctcgtcggagacggacgtccctgcttctcgatggtgagcctgaccagctccttcactccatccagcacagccttgatgacccccttcacagtcgtcaccatctccttgtcttctgagttcacgccttccagcatcacttggtcagaccagcgaatgaggttggcgaggctttggtacactcggctatagcaggaagagagggctgagctgtgctgaattcgaggatcgttctgcaccaggggtaagatggcctccagcaccttgctggctgaccctggaagcatctccagtaccttcttatcaattgccattttgtccacaatggtcttaaagtagcgcagggcactgacaacttccttctctttctcctccagccagctcaggtttttgttcacaggcttctctggaatctttacggacacctcagctggttttcccttctttgatggcgttctcttgattttgggtgagtggaatttgtccatcagcttcatggtgaaggaagagagatgagaacgctgagagtagagtttgtgtgatgatctaactaacatccaagggaactggctgagaagaaagaacacccagtcaaatcacagatgtgtaggatgtgagaactggaaaggaaggccctttcgcatcaacctcttcattctttaagaaactgcaacaagtgacatgtgcaaggctctggagttggcagcggtgactgaa

SEQ ID NO: 16457 - RNA, 4609 nt, Homo sapiens
  source 1..4609: mol_type = other RNA
gtcctaggaggctcctctgtggccaggcttctgcctccctgcaccctgagggaccattcgggtgcctcagggatgcccttccctcccaggggcactgacagcactggctgaaaggtctgaagagccagaggaggagccctgctggctggcccaggatggggcaaggagggagggaaagccaggggatggggagggacatgagatggagtttaaggcacacagcgagcgatggaggagggaggtgctggcctctcccctctgaattaactcccccaggagctcagctctggcctcagtttggtgaggttcagaagactcccagcaataaaaagtatttcttggatgatcaagtcctcccttactccagcctcctcttctcagctccccaggtggtgtgggaggggcccagtggcctggggtggggggtaaggggcgacgggatgacagagactgctgctgctctcaggcgggcaagggaggccctgatggcgccagtaccgcggggcagagcaccagctgcggggctgctaaggcgtcacctgcgtacctttccgggcctgctgaaaagctcacaccatcctccatgcatcagaaggggaagcggaaagtgaaaggatcctcccccgagtctactctgcattctgcccacccagctgcttgcccccattccagggcccctgcaggacaggccaccccaggaggcctccactcatttgagatttcagaagattcagggaccctggagcttagggagggggagcacccaccacttccttggtctgctgatgaggtctctgctgctctctccctggaggggagtgggtggaaggtcaagaggggagagatggaagtaaaagcagaaaacaaaaccaaaccagaaaaccaccggtttgtaaattggcaacaagacctgcctgctggctgccctgaggcccacgggtctgctcccacagaggaaggaggcaggaagcggctggcaggctccagctcccgcccggccccgctgagggctggccagcctcatggctccgaggccgggactcctgccatgcgcctaacaggtccaaggtcctctccggtctgggagctgccctctgcgcccctcgagcattctcctggatcccggcgtctgctcctaggtcttctcttcccggtctgtttttctccttgttatgttcctgggtttaattttcagagacagttcccatagggcctcctcagccaggtggtcactgaagtcattgaagaagtttataatgtcgtcgttcctccgcatgtcatagtgcgcctgctggaagcagcgcatgctgtcgaggatgttgaactgctgccaccgcttggagaagttcactttcccgtcgatgtagtctgggtttcccaggtgaacgaaggtcaggtcctgcaggatcagccccaggtacgggatgcacggcggttccacctccgagagggcggcccggtaggctcggaaggaggacgagctgtcgatcagtgtgcagtactcggccaggccctctgaagtctgcttctgccactccagcctgcggatgggcgccgagtccagggcagagaggatggccaagtaggagttgaagttattcagcttccgcaagtgcttcatgatcttgatgaacttcaagagcagccgttccctgtcctgggccttttcctgtaacatgattatggaccggacccagtaggacatgttgttgaagtgctccgtgaactgggtcaagttggggctcttctcctcattctgctcttttgcccaaagcaaaacctcaggaatctctattttatagaagagctcagcatccagcagcgttagctgctccgctatctcatggctgtgaaagtcgtgcaaggtccccggcctggctgctaccccccgggctgccaggggctggctggaggtggcacacctgagtagcttcttctggtccaccttgtccaggatgttcttccggagcacacgggccaggctcagctccccattgcacaccaggcggaagaccagttccatcagcagcttcaggatctcttctgtcaactccaccaggcagagctcatccaccacccgtaccagcacgaagaacgtgttcttgctgacgcgcttcttgaatgtgtcggcaaagggagagaatttctcatatctgtactgcagcttcttgatgagctcctctggggagatgaaggtcctgtaggtggtcaggaatgcctcgcagtacaacaccaaatctttcctgtcagtctcagtagcatggaccagtaagatgtccccagatcctccgcggacgtccggcccgtcatcaccctcctgcttgagcgtcagcctggacataatttcgttgtggtcaatgagggacagctcgtccacttcctcctccgactgagccgactccagagcatctggtgactttggggccctctcactgccgtctctgctgtccttcccagggacgccgctgaccgctgagggatctctgggatgtccgtctttcccagccggtggctctcctcgagagggagccagctcctcgctgctctggccagaggaatacagattgacatattcaccctcaccagcttcctcactggcgttttcactcagctgccgctgcttggggggtagggcgggcggcggggccagctcctgcacggagtccaccccactgaaggagtcgctgaagccgtatacctccatgaggagcttgttcttctgctggtagatgtgctcgttctgtggcgtctggtagaacatagagggctgcggctccgagtagtcctccagcaactgcatgtaggccagcatgtgtttgtttttcttctctggtagaggaggtggtttttctgggtcaccggttgactcaggagcagtaaaatcacccacaaattcgacaggggctgaggaacctccatgctgaaagggcagaatagcagcaaagggcgcgtaggggacggatgggatcggggctgtgctctgcaggtcctccccagagatgttgtcatactgcgagggatgccgctcgtaggacaccctgcagccagagccgtccgccgtctgggaggctgcgctcctgcgcttcttctcggggagagcaggtggcgtatctgtctgctgccctggggccagaggtccgtctggctggggatggccgccaagaggcagctggaaaggagggccaagaaatggagacccagactcccccaaagactctggcaacgggctaaggttccaggccgtctgctgaggtatctggtctgcgttagagaggtcttgctggaggaattcatagtcgggatcatagtggtctagtgtttcacagcttgtgttccgggagcactgcccactgtccctgtccagagaggacagctgctcgtctgacttgctgagcttgcctatgctgctgcagggggagaggcggggcgactctccaccatatgagtggctgcctcctgacagtcgcctctgtgcgtaacagtcaacatcaaaatcctgcctattgattccaacaggcaaactggagccactggtggctcggctcatgggggccaccacagccactcgggtaggggacggcgccgactgtcttttcttgggtggcaatgctggtggaggactattatcaaccacccgaatgccaggcagaggaggcttggggggcgcgacctcttcatccgtggcatctgggaggagctcagttgactgtgacatcccagtcgtcttgtttaggatctctacctcgcggtctgtcagggggagctctgctgggccatcaggcttgctggcaggggaactgggcttcacggggctcgtcggagacggacgtccctgcttctcgatggtgagcctgaccagctccttcactccatccagcacagccttgatgacccccttcacagtcgtcaccatctccttgtcttctgagttcacgccttccagcatcacttggtcagaccagcgaatgaggttggcgaggctttggtacactcggctatagcaggaagagagggctgagctgtgctgaattcgaggatcgttctgcaccaggggtaagatggcctccagcaccttgctggctgaccctggaagcatctccagtaccttcttatcaattgccattttgtccacaatggtcttaaagtagcgcagggcactgacaacttccttctctttctcctccagccagctcaggtttttgttcacaggcttctctggaatctttacggacacctcagctggttttcccttctttgatggcgttctcttgattttgggtgagtggaatttgtccatcagcttcatggtgaaggaagagagatgagaacgctgagagtctggaacgacacctcctgtcctcttgttctgttccaaggttgtcaggctgggacgaaatcccaagaaagaaatgggcatgtggtcactatcatagcagactgccagttagggacatcagaatatatttctctgtcctcaagttaggaagtgagaggacaaacctggccttctgtgttgtttcagccactaattggttttgtcaattaggcaaaacataatttctctaagcctcttttctcatccacaggcattagcctagtcagcggttct

SEQ ID NO: 16458 - RNA, 4890 nt, Homo sapiens
  source 1..4890: mol_type = other RNA
gtcctaggaggctcctctgtggccaggcttctgcctccctgcaccctgagggaccattcgggtgcctcagggatgcccttccctcccaggggcactgacagcactggctgaaaggtctgaagagccagaggaggagccctgctggctggcccaggatggggcaaggagggagggaaagccaggggatggggagggacatgagatggagtttaaggcacacagcgagcgatggaggagggaggtgctggcctctcccctctgaattaactcccccaggagctcagctctggcctcagtttggtgaggttcagaagactcccagcaataaaaagtatttcttggatgatcaagtcctcccttactccagcctcctcttctcagctccccaggtggtgtgggaggggcccagtggcctggggtggggggtaaggggcgacgggatgacagagactgctgctgctctcaggcgggcaagggaggccctgatggcgccagtaccgcggggcagagcaccagctgcggggctgctaaggcgtcacctgcgtacctttccgggcctgctgaaaagctcacaccatcctccatgcatcagaaggggaagcggaaagtgaaaggatcctcccccgagtctactctgcattctgcccacccagctgcttgcccccattccagggcccctgcaggacaggccaccccaggaggcctccactcatttgagatttcagaagattcagggaccctggagcttagggagggggagcacccaccacttccttggtctgctgatgaggtctctgctgctctctccctggaggggagtgggtggaaggtcaagaggggagagatggaagtaaaagcagaaaacaaaaccaaaccagaaaaccaccggtttgtaaattggcaacaagacctgcctgctggctgccctgaggcccacgggtctgctcccacagaggaaggaggcaggaagcggctggcaggctccagctcccgcccggccccgctgagggctggccagcctcatggctccgaggccgggactcctgccatgcgcctaacaggtccaaggtcctctccggtctgggagctgccctctgcgcccctcgagcattctcctggatcccggcgtctgctcctaggtcttctcttcccggtctgtttttctccttgttatgttcctgggtttaattttcagagacagttcccatagggcctcctcagccaggtggtcactgaagtcattgaagaagtttataatgtcgtcgttcctccgcatgtcatagtgcgcctgctggaagcagcgcatgctgtcgaggatgttgaactgctgccaccgcttggagaagttcactttcccgtcgatgtagtctgggtttcccaggtgaacgaaggtcaggtcctgcaggatcagccccaggtacgggatgcacggcggttccacctccgagagggcggcccggtaggctcggaaggaggacgagctgtcgatcagtgtgcagtactcggccaggccctctgaagtctgcttctgccactccagcctgcggatgggcgccgagtccagggcagagaggatggccaagtaggagttgaagttattcagcttccgcaagtgcttcatgatcttgatgaacttcaagagcagccgttccctgtcctgggccttttcctgtaacatgattatggaccggacccagtaggacatgttgttgaagtgctccgtgaactgggtcaagttggggctcttctcctcattctgctcttttgcccaaagcaaaacctcaggaatctctattttatagaagagctcagcatccagcagcgttagctgctccgctatctcatggctgtgaaagtcgtgcaaggtccccggcctggctgctaccccccgggctgccaggggctggctggaggtggcacacctgagtagcttcttctggtccaccttgtccaggatgttcttccggagcacacgggccaggctcagctccccattgcacaccaggcggaagaccagttccatcagcagcttcaggatctcttctgtcaactccaccaggcagagctcatccaccacccgtaccagcacgaagaacgtgttcttgctgacgcgcttcttgaatgtgtcggcaaagggagagaatttctcatatctgtactgcagcttcttgatgagctcctctggggagatgaaggtcctgtaggtggtcaggaatgcctcgcagtacaacaccaaatctttcctgtcagtctcagtagcatggaccagtaagatgtccccagatcctccgcggacgtccggcccgtcatcaccctcctgcttgagcgtcagcctggacataatttcgttgtggtcaatgagggacagctcgtccacttcctcctccgactgagccgactccagagcatctggtgactttggggccctctcactgccgtctctgctgtccttcccagggacgccgctgaccgctgagggatctctgggatgtccgtctttcccagccggtggctctcctcgagagggagccagctcctcgctgctctggccagaggaatacagattgacatattcaccctcaccagcttcctcactggcgttttcactcgagggcacgggcaagctgccgtgccggctgagaaaggagttagagacggacacactgaggccctgagcggcactgccgtcctcgggggtgaaggccactttagtttgctggacacagtgggagacagaggagaaggaagaagcagcacaggaggcctgcagctgccgctgcttggggggtagggcgggcggcggggccagctcctgcacggagtccaccccactgaaggagtcgctgaagccgtatacctccatgaggagcttgttcttctgctggtagatgtgctcgttctgtggcgtctggtagaacatagagggctgcggctccgagtagtcctccagcaactgcatgtaggccagcatgtgtttgtttttcttctctggtagaggaggtggtttttctgggtcaccggttgactcaggagcagtaaaatcacccacaaattcgacaggggctgaggaacctccatgctgaaagggcagaatagcagcaaagggcgcgtaggggacggatgggatcggggctgtgctctgcaggtcctccccagagatgttgtcatactgcgagggatgccgctcgtaggacaccctgcagccagagccgtccgccgtctgggaggctgcgctcctgcgcttcttctcggggagagcaggtggcgtatctgtctgctgccctggggccagaggtccgtctggctggggatggccgccaagaggcagctggaaaggagggccaagaaatggagacccagactcccccaaagactctggcaacgggctaaggttccaggccgtctgctgaggtatctggtctgcgttagagaggtcttgctggaggaattcatagtcgggatcatagtggtctagtgtttcacagcttgtgttccgggagcactgcccactgtccctgtccagagaggacagctgctcgtctgacttgctgagcttgcctatgctgctgcagggggagaggcggggcgactctccaccatatgagtggctgcctcctgacagtcgcctctgtgcgtaacagtcaacatcaaaatcctgcctattgattccaacaggcaaactggagccactggtggctcggctcatgggggccaccacagccactcgggtaggggacggcgccgactgtcttttcttgggtggcaatgctggtggaggactattatcaaccacccgaatgccaggcagaggaggcttggggggcgcgacctcttcatccgtggcatctgggaggagctcagttgactgtgacatcccagtcgtcttgtttaggatctctacctcgcggtctgtcagggggagctctgctgggccatcaggcttgctggcaggggaactgggcttcacggggctcgtcggagacggacgtccctgcttctcgatggtgagcctgaccagctccttcactccatccagcacagccttgatgacccccttcacagtcgtcaccatctccttgtcttctgagttcacgccttccagcatcacttggtcagaccagcgaatgaggttggcgaggctttggtacactcggctatagcaggaagagagggctgagctgtgctgaattcgaggatcgttctgcaccaggggtaagatggcctccagcaccttgctggctgaccctggaagcatctccagtaccttcttatcaattgccattttgtccacaatggtcttaaagtagcgcagggcactgacaacttccttctctttctcctccagccagctcaggttcttctgcctttgagacctggaagccacagcactggtggacataaattctactgcctgctgctccagatccaaggggagagggtagccctctggtagaaatctgtctgttgcctcctggaagagaggaaacctggattctttgttcacaggcttctctggaatctttacggacacctcagctggttttcccttctttgatggcgttctcttgattttgggtgagtggaatttgtccatcagcttcatggtgaaggaagagagatgagaacgctgagagtctggaacgacacctcctgtcctcttgttctgttccaaggttgtcaggctgggacgaaatcccaagaaagaaatgggcatgtggtcactatcatagcagactgccagttagggacatcagaatatatttctctgtcctcaagttaggaagtgagaggacaaacctggccttctgtgttgtttcagccactaattggttttgtcaattaggcaaaacataatttctctaagcctcttttctcatccacaggcattag

SEQ ID NO: 16459 - RNA, 4989 nt, Homo sapiens
  source 1..4989: mol_type = other RNA
gtcctaggaggctcctctgtggccaggcttctgcctccctgcaccctgagggaccattcgggtgcctcagggatgcccttccctcccaggggcactgacagcactggctgaaaggtctgaagagccagaggaggagccctgctggctggcccaggatggggcaaggagggagggaaagccaggggatggggagggacatgagatggagtttaaggcacacagcgagcgatggaggagggaggtgctggcctctcccctctgaattaactcccccaggagctcagctctggcctcagtttggtgaggttcagaagactcccagcaataaaaagtatttcttggatgatcaagtcctcccttactccagcctcctcttctcagctccccaggtggtgtgggaggggcccagtggcctggggtggggggtaaggggcgacgggatgacagagactgctgctgctctcaggcgggcaagggaggccctgatggcgccagtaccgcggggcagagcaccagctgcggggctgctaaggcgtcacctgcgtacctttccgggcctgctgaaaagctcacaccatcctccatgcatcagaaggggaagcggaaagtgaaaggatcctcccccgagtctactctgcattctgcccacccagctgcttgcccccattccagggcccctgcaggacaggccaccccaggaggcctccactcatttgagatttcagaagattcagggaccctggagcttagggagggggagcacccaccacttccttggtctgctgatgaggtctctgctgctctctccctggaggggagtgggtggaaggtcaagaggggagagatggaagtaaaagcagaaaacaaaaccaaaccagaaaaccaccggtttgtaaattggcaacaagacctgcctgctggctgccctgaggcccacgggtctgctcccacagaggaaggaggcaggaagcggctggcaggctccagctcccgcccggccccgctgagggctggccagcctcatggctccgaggccgggactcctgccatgcgcctaacaggtccaaggtcctctccggtctgggagctgccctctgcgcccctcgagcattctcctggatcccggcgtctgctcctaggtcttctcttcccggtctgtttttctccttgttatgttcctgggtttaattttcagagacagttcccatagggcctcctcagccaggtggtcactgaagtcattgaagaagtttataatgtcgtcgttcctccgcatgtcatagtgcgcctgctggaagcagcgcatgctgtcgaggatgttgaactgctgccaccgcttggagaagttcactttcccgtcgatgtagtctgggtttcccaggtgaacgaaggtcaggtcctgcaggatcagccccaggtacgggatgcacggcggttccacctccgagagggcggcccggtaggctcggaaggaggacgagctgtcgatcagtgtgcagtactcggccaggccctctgaagtctgcttctgccactccagcctgcggatgggcgccgagtccagggcagagaggatggccaagtaggagttgaagttattcagcttccgcaagtgcttcatgatcttgatgaacttcaagagcagccgttccctgtcctgggccttttcctgtaacatgattatggaccggacccagtaggacatgttgttgaagtgctccgtgaactgggtcaagttggggctcttctcctcattctgctcttttgcccaaagcaaaacctcaggaatctctattttatagaagagctcagcatccagcagcgttagctgctccgctatctcatggctgtgaaagtcgtgcaaggtccccggcctggctgctaccccccgggctgccaggggctggctggaggtggcacacctgagtagcttcttctggtccaccttgtccaggatgttcttccggagcacacgggccaggctcagctccccattgcacaccaggcggaagaccagttccatcagcagcttcaggatctcttctgtcaactccaccaggcagagctcatccaccacccgtaccagcacgaagaacgtgttcttgctgacgcgcttcttgaatgtgtcggcaaagggagagaatttctcatatctgtactgcagcttcttgatgagctcctctggggagatgaaggtcctgtaggtggtcaggaatgcctcgcagtacaacaccaaatctttcctgtcagtctcagtagcatggaccagtaagatgtccccagatcctccgcggacgtccggcccgtcatcaccctcctgcttgagcgtcagcctggacataatttcgttgtggtcaatgagggacagctcgtccacttcctcctccgactgagccgactccagagcatctggtgactttggggccctctcactgccgtctctgctgtccttcccagggacgccgctgaccgctgagggatctctgggatgtccgtctttcccagccggtggctctcctcgagagggagccagctcctcgctgctctggccagaggaatacagattgacatattcaccctcaccagcttcctcactggcgttttcactcgagtcagtgaaagaggtttcggaaggaaggcagacagtattcccatgaaagctgctctcctgagaagccgagagaggcccgtccacggtgctgggaggtggaccggccatggttggcacggctaagtcagagctctgagactggtgggcaggtgggaaatgtggagaggaagaggaggtaggcggaaggaaaggcggaacggaagcttggtggtgaggcacgaaatcctgggagtaggacctaaacacagacttatacagctgccgctgcttggggggtagggcgggcggcggggccagctcctgcacggagtccaccccactgaaggagtcgctgaagccgtatacctccatgaggagcttgttcttctgctggtagatgtgctcgttctgtggcgtctggtagaacatagagggctgcggctccgagtagtcctccagcaactgcatgtaggccagcatgtgtttgtttttcttctctggtagaggaggtggtttttctgggtcaccggttgactcaggagcagtaaaatcacccacaaattcgacaggggctgaggaacctccatgctgaaagggcagaatagcagcaaagggcgcgtaggggacggatgggatcggggctgtgctctgcaggtcctccccagagatgttgtcatactgcgagggatgccgctcgtaggacaccctgcagccagagccgtccgccgtctgggaggctgcgctcctgcgcttcttctcggggagagcaggtggcgtatctgtctgctgccctggggccagaggtccgtctggctggggatggccgccaagaggcagctggaaaggagggccaagaaatggagacccagactcccccaaagactctggcaacgggctaaggttccaggccgtctgctgaggtatctggtctgcgttagagaggtcttgctggaggaattcatagtcgggatcatagtggtctagtgtttcacagcttgtgttccgggagcactgcccactgtccctgtccagagaggacagctgctcgtctgacttgctgagcttgcctatgctgctgcagggggagaggcggggcgactctccaccatatgagtggctgcctcctgacagtcgcctctgtgcgtaacagtcaacatcaaaatcctgcctattgattccaacaggcaaactggagccactggtggctcggctcatgggggccaccacagccactcgggtaggggacggcgccgactgtcttttcttgggtggcaatgctggtggaggactattatcaaccacccgaatgccaggcagaggaggcttggggggcgcgacctcttcatccgtggcatctgggaggagctcagttgactgtgacatcccagtcgtcttgtttaggatctctacctcgcggtctgtcagggggagctctgctgggccatcaggcttgctggcaggggaactgggcttcacggggctcgtcggagacggacgtccctgcttctcgatggtgagcctgaccagctccttcactccatccagcacagccttgatgacccccttcacagtcgtcaccatctccttgtcttctgagttcacgccttccagcatcacttggtcagaccagcgaatgaggttggcgaggctttggtacactcggctatagcaggaagagagggctgagctgtgctgaattcgaggatcgttctgcaccaggggtaagatggcctccagcaccttgctggctgaccctggaagcatctccagtaccttcttatcaattgccattttgtccacaatggtcttaaagtagcgcagggcactgacaacttccttctctttctcctccagccagctcaggttcttctgcctttgagacctggaagccacagcactggtggacataaattctactgcctgctgctccagatccaaggggagagggtagccctctggtagaaatctgtctgttgcctcctggaagagaggaaacctggattctttgttcacaggcttctctggaatctttacggacacctcagctggttttcccttctttgatggcgttctcttgattttgggtgagtggaatttgtccatcagcttcatggtgaaggaagagagatgagaacgctgagagtctggaacgacacctcctgtcctcttgttctgttccaaggttgtcaggctgggacgaaatcccaagaaagaaatgggcatgtggtcactatcatagcagactgccagttagggacatcagaatatatttctctgtcctcaagttaggaagtgagaggacaaacctggccttctgtgttgtttcagccactaattggttttgtcaattaggcaaaacataatttctctaagcctcttttctcatccacaggcattag

SEQ ID NO: 16460 - RNA, 5145 nt, Homo sapiens
  source 1..5145: mol_type = other RNA
gtcctaggaggctcctctgtggccaggcttctgcctccctgcaccctgagggaccattcgggtgcctcagggatgcccttccctcccaggggcactgacagcactggctgaaaggtctgaagagccagaggaggagccctgctggctggcccaggatggggcaaggagggagggaaagccaggggatggggagggacatgagatggagtttaaggcacacagcgagcgatggaggagggaggtgctggcctctcccctctgaattaactcccccaggagctcagctctggcctcagtttggtgaggttcagaagactcccagcaataaaaagtatttcttggatgatcaagtcctcccttactccagcctcctcttctcagctccccaggtggtgtgggaggggcccagtggcctggggtggggggtaaggggcgacgggatgacagagactgctgctgctctcaggcgggcaagggaggccctgatggcgccagtaccgcggggcagagcaccagctgcggggctgctaaggcgtcacctgcgtacctttccgggcctgctgaaaagctcacaccatcctccatgcatcagaaggggaagcggaaagtgaaaggatcctcccccgagtctactctgcattctgcccacccagctgcttgcccccattccagggcccctgcaggacaggccaccccaggaggcctccactcatttgagatttcagaagattcagggaccctggagcttagggagggggagcacccaccacttccttggtctgctgatgaggtctctgctgctctctccctggaggggagtgggtggaaggtcaagaggggagagatggaagtaaaagcagaaaacaaaaccaaaccagaaaaccaccggtttgtaaattggcaacaagacctgcctgctggctgccctgaggcccacgggtctgctcccacagaggaaggaggcaggaagcggctggcaggctccagctcccgcccggccccgctgagggctggccagcctcatggctccgaggccgggactcctgccatgcgcctaacaggtccaaggtcctctccggtctgggagctgccctctgcgcccctcgagcattctcctggatcccggcgtctgctcctaggtcttctcttcccggtctgtttttctccttgttatgttcctgggtttaattttcagagacagttcccatagggcctcctcagccaggtggtcactgaagtcattgaagaagtttataatgtcgtcgttcctccgcatgtcatagtgcgcctgctggaagcagcgcatgctgtcgaggatgttgaactgctgccaccgcttggagaagttcactttcccgtcgatgtagtctgggtttcccaggtgaacgaaggtcaggtcctgcaggatcagccccaggtacgggatgcacggcggttccacctccgagagggcggcccggtaggctcggaaggaggacgagctgtcgatcagtgtgcagtactcggccaggccctctgaagtctgcttctgccactccagcctgcggatgggcgccgagtccagggcagagaggatggccaagtaggagttgaagttattcagcttccgcaagtgcttcatgatcttgatgaacttcaagagcagccgttccctgtcctgggccttttcctgtaacatgattatggaccggacccagtaggacatgttgttgaagtgctccgtgaactgggtcaagttggggctcttctcctcattctgctcttttgcccaaagcaaaacctcaggaatctctattttatagaagagctcagcatccagcagcgttagctgctccgctatctcatggctgtgaaagtcgtgcaaggtccccggcctggctgctaccccccgggctgccaggggctggctggaggtggcacacctgagtagcttcttctggtccaccttgtccaggatgttcttccggagcacacgggccaggctcagctccccattgcacaccaggcggaagaccagttccatcagcagcttcaggatctcttctgtcaactccaccaggcagagctcatccaccacccgtaccagcacgaagaacgtgttcttgctgacgcgcttcttgaatgtgtcggcaaagggagagaatttctcatatctgtactgcagcttcttgatgagctcctctggggagatgaaggtcctgtaggtggtcaggaatgcctcgcagtacaacaccaaatctttcctgtcagtctcagtagcatggaccagtaagatgtccccagatcctccgcggacgtccggcccgtcatcaccctcctgcttgagcgtcagcctggacataatttcgttgtggtcaatgagggacagctcgtccacttcctcctccgactgagccgactccagagcatctggtgactttggggccctctcactgccgtctctgctgtccttcccagggacgccgctgaccgctgagggatctctgggatgtccgtctttcccagccggtggctctcctcgagagggagccagctcctcgctgctctggccagaggaatacagattgacatattcaccctcaccagcttcctcactggcgttttcactcgagtcagtgaaagaggtttcggaaggaaggcagacagtattcccatgaaagctgctctcctgagaagccgagagaggcccgtccacggtgctgggaggtggaccggccatggttggcacggctaagtcagagctctgagactggtgggcaggtgggaaatgtggagaggaagaggaggtaggcggaaggaaaggcggaacggaagcttggtggtgaggcacgaaatcctgggagtaggacctaaacacagacttatacgagggcacgggcaagctgccgtgccggctgagaaaggagttagagacggacacactgaggccctgagcggcactgccgtcctcgggggtgaaggccactttagtttgctggacacagtgggagacagaggagaaggaagaagcagcacaggaggccagctgccgctgcttggggggtagggcgggcggcggggccagctcctgcacggagtccaccccactgaaggagtcgctgaagccgtatacctccatgaggagcttgttcttctgctggtagatgtgctcgttctgtggcgtctggtagaacatagagggctgcggctccgagtagtcctccagcaactgcatgtaggccagcatgtgtttgtttttcttctctggtagaggaggtggtttttctgggtcaccggttgactcaggagcagtaaaatcacccacaaattcgacaggggctgaggaacctccatgctgaaagggcagaatagcagcaaagggcgcgtaggggacggatgggatcggggctgtgctctgcaggtcctccccagagatgttgtcatactgcgagggatgccgctcgtaggacaccctgcagccagagccgtccgccgtctgggaggctgcgctcctgcgcttcttctcggggagagcaggtggcgtatctgtctgctgccctggggccagaggtccgtctggctggggatggccgccaagaggcagctggaaaggagggccaagaaatggagacccagactcccccaaagactctggcaacgggctaaggttccaggccgtctgctgaggtatctggtctgcgttagagaggtcttgctggaggaattcatagtcgggatcatagtggtctagtgtttcacagcttgtgttccgggagcactgcccactgtccctgtccagagaggacagctgctcgtctgacttgctgagcttgcctatgctgctgcagggggagaggcggggcgactctccaccatatgagtggctgcctcctgacagtcgcctctgtgcgtaacagtcaacatcaaaatcctgcctattgattccaacaggcaaactggagccactggtggctcggctcatgggggccaccacagccactcgggtaggggacggcgccgactgtcttttcttgggtggcaatgctggtggaggactattatcaaccacccgaatgccaggcagaggaggcttggggggcgcgacctcttcatccgtggcatctgggaggagctcagttgactgtgacatcccagtcgtcttgtttaggatctctacctcgcggtctgtcagggggagctctgctgggccatcaggcttgctggcaggggaactgggcttcacggggctcgtcggagacggacgtccctgcttctcgatggtgagcctgaccagctccttcactccatccagcacagccttgatgacccccttcacagtcgtcaccatctccttgtcttctgagttcacgccttccagcatcacttggtcagaccagcgaatgaggttggcgaggctttggtacactcggctatagcaggaagagagggctgagctgtgctgaattcgaggatcgttctgcaccaggggtaagatggcctccagcaccttgctggctgaccctggaagcatctccagtaccttcttatcaattgccattttgtccacaatggtcttaaagtagcgcagggcactgacaacttccttctctttctcctccagccagctcaggttcttctgcctttgagacctggaagccacagcactggtggacataaattctactgcctgctgctccagatccaaggggagagggtagccctctggtagaaatctgtctgttgcctcctggaagagaggaaacctggattctttgttcacaggcttctctggaatctttacggacacctcagctggttttcccttctttgatggcgttctcttgattttgggtgagtggaatttgtccatcagcttcatggtgaaggaagagagatgagaacgctgagagtctggaacgacacctcctgtcctcttgttctgttccaaggttgtcaggctgggacgaaatcccaagaaagaaatgggcatgtggtcactatcatagcagactgccagttagggacatcagaatatatttctctgtcctcaagttaggaagtgagaggacaaacctggccttctgtgttgtttcagccactaattggttttgtcaattaggcaaaacataatttctctaagcctcttttctcatccacaggcattag

SEQ ID NO: 16461 - RNA, 5173 nt, Homo sapiens
  source 1..5173: mol_type = other RNA
gtcctaggaggctcctctgtggccaggcttctgcctccctgcaccctgagggaccattcgggtgcctcagggatgcccttccctcccaggggcactgacagcactggctgaaaggtctgaagagccagaggaggagccctgctggctggcccaggatggggcaaggagggagggaaagccaggggatggggagggacatgagatggagtttaaggcacacagcgagcgatggaggagggaggtgctggcctctcccctctgaattaactcccccaggagctcagctctggcctcagtttggtgaggttcagaagactcccagcaataaaaagtatttcttggatgatcaagtcctcccttactccagcctcctcttctcagctccccaggtggtgtgggaggggcccagtggcctggggtggggggtaaggggcgacgggatgacagagactgctgctgctctcaggcgggcaagggaggccctgatggcgccagtaccgcggggcagagcaccagctgcggggctgctaaggcgtcacctgcgtacctttccgggcctgctgaaaagctcacaccatcctccatgcatcagaaggggaagcggaaagtgaaaggatcctcccccgagtctactctgcattctgcccacccagctgcttgcccccattccagggcccctgcaggacaggccaccccaggaggcctccactcatttgagatttcagaagattcagggaccctggagcttagggagggggagcacccaccacttccttggtctgctgatgaggtctctgctgctctctccctggaggggagtgggtggaaggtcaagaggggagagatggaagtaaaagcagaaaacaaaaccaaaccagaaaaccaccggtttgtaaattggcaacaagacctgcctgctggctgccctgaggcccacgggtctgctcccacagaggaaggaggcaggaagcggctggcaggctccagctcccgcccggccccgctgagggctggccagcctcatggctccgaggccgggactcctgccatgcgcctaacaggtccaaggtcctctccggtctgggagctgccctctgcgcccctcgagcattctcctggatcccggcgtctgctcctaggtcttctcttcccggtctgtttttctccttgttatgttcctgggtttaattttcagagacagttcccatagggcctcctcagccaggtggtcactgaagtcattgaagaagtttataatgtcgtcgttcctccgcatgtcatagtgcgcctgctggaagcagcgcatgctgtcgaggatgttgaactgctgccaccgcttggagaagttcactttcccgtcgatgtagtctgggtttcccaggtgaacgaaggtcaggtcctgcaggatcagccccaggtacgggatgcacggcggttccacctccgagagggcggcccggtaggctcggaaggaggacgagctgtcgatcagtgtgcagtactcggccaggccctctgaagtctgcttctgccactccagcctgcggatgggcgccgagtccagggcagagaggatggccaagtaggagttgaagttattcagcttccgcaagtgcttcatgatcttgatgaacttcaagagcagccgttccctgtcctgggccttttcctgtaacatgattatggaccggacccagtaggacatgttgttgaagtgctccgtgaactgggtcaagttggggctcttctcctcattctgctcttttgcccaaagcaaaacctcaggaatctctattttatagaagagctcagcatccagcagcgttagctgctccgctatctcatggctgtgaaagtcgtgcaaggtccccggcctggctgctaccccccgggctgccaggggctggctggaggtggcacacctgagtagcttcttctggtccaccttgtccaggatgttcttccggagcacacgggccaggctcagctccccattgcacaccaggcggaagaccagttccatcagcagcttcaggatctcttctgtcaactccaccaggcagagctcatccaccacccgtaccagcacgaagaacgtgttcttgctgacgcgcttcttgaatgtgtcggcaaagggagagaatttctcatatctgtactgcagcttcttgatgagctcctctggggagatgaaggtcctgtaggtggtcaggaatgcctcgcagtacaacaccaaatctttcctgtcagtctcagtagcatggaccagtaagatgtccccagatcctccgcggacgtccggcccgtcatcaccctcctgcttgagcgtcagcctggacataatttcgttgtggtcaatgagggacagctcgtccacttcctcctccgactgagccgactccagagcatctggtgactttggggccctctcactgccgtctctgctgtccttcccagggacgccgctgaccgctgagggatctctgggatgtccgtctttcccagccggtggctctcctcgagagggagccagctcctcgctgctctggccagaggaatacagattgacatattcaccctcaccagcttcctcactggcgttttcactcgagtcagtgaaagaggtttcggaaggaaggcagacagtattcccatgaaagctgctctcctgagaagccgagagaggcccgtccacggtgctgggaggtggaccggccatggttggcacggctaagtcagagctctgagactggtgggcaggtgggaaatgtggagaggaagaggaggtaggcggaaggaaaggcggaacggaagcttggtggtgaggcacgaaatcctgggagtaggacctaaacacagacttatacgagggcacgggcaagctgccgtgccggctgagaaaggagttagagacggacacactgaggccctgagcggcactgccgtcctcgggggtgaaggccactttagtttgctggacacagtgggagacagaggagaaggaagaagcagcacaggaggccagctgccgctgcttggggggtagggcgggcggcggggccagctcctgcacggagtccaccccactgaaggagtcgctgaagccgtatacctccatgaggagcttgttcttctgctggtagatgtgctcgttctgtggcgtctggtagaacatagagggctgcggctccgagtagtcctccagcaactgcatgtaggccagcatgtgtttgtttttcttctctggtagaggaggtggtttttctgggtcaccggttgactcaggagcagtaaaatcacccacaaattcgacaggggctgaggaacctccatgctgaaagggcagaatagcagcaaagggcgcgtaggggacggatgggatcggggctgtgctctgcaggtcctccccagagatgttgtcatactgcgagggatgccgctcgtaggacaccctgcagccagagccgtccgccgtctgggaggctgcgctcctgcgcttcttctcggggagagcaggtggcgtatctgtctgctgccctggggccagaggtccgtctggctggggatggccgccaagaggcagctggaaaggagggccaagaaatggagacccagactcccccaaagactctggcaacgggctaaggttccaggccgtctgctgaggtatctggtctgcgttagagaggtcttgctggaggaattcatagtcgggatcatagtggtctagtgtttcacagcttgtgttccgggagcactgcccactgtccctgtccagagaggacagctgctcgtctgacttgctgagcttgcctatgctgctgcagggggagaggcggggcgactctccaccatatgagtggctgcctcctgacagtcgcctctgtgcgtaacagtcaacatcaaaatcctgcctattgattccaacaggcaaactggagccactggtggctcggctcatgggggccaccacagccactcgggtaggggacggcgccgactgtcttttcttgggtggcaatgctggtggaggactattatcaaccacccgaatgccaggcagaggaggcttggggggcgcgacctcttcatccgtggcatctgggaggagctcagttgactgtgacatcccagtcgtcttgtttaggatctctacctcgcggtctgtcagggggagctctgctgggccatcaggcttgctggcaggggaactgggcttcacggggctcgtcggagacggacgtccctgcttctcgatggtgagcctgaccagctccttcactccatccagcacagccttgatgacccccttcacagtcgtcaccatctccttgtcttctgagttcacgccttccagcatcacttggtcagaccagcgaatgaggttggcgaggctttggtacactcggctatagcaggaagagagggctgagctgtgctgaattcgaggatcgttctgcaccaggggtaagatggcctccagcaccttgctggctgaccctggaagcatctccagtaccttcttatcaattgccattttgtccacaatggtcttaaagtagcgcagggcactgacaacttccttctctttctcctccagccagctcaggttcttctgcctttgagacctggaagccacagcactggtggacataaattctactgcctgctgctccagatccaaggggagagggtagccctctggtagaaatctgtctgttgcctctttgttcacaggcttctctggaatctttacggacacctcagctggttttcccttctttgatggcgttctcttgattttgggtgagtggaatttgtccatcagcttcatggtgaaggaagagagatgagaacgctgagagtctgctttctcgatcttgccggacatttccgggctgcgccggaggccgaggccgccgctcatcgggcccgggccgggccgccgcggggcgacaggggcggcgcgcccgccgctcgcctcggccctggctcgccacgcctcagacccgcgccggcatggcgggctccgcgcggccgcggccctgcgctcggcgaccgcgctccagcccgcccgggcccagccgctcccgccgcgcccgccgccgccgctccgcctcccgcgcgcccgccgccgctcccccggcccgcgagccggccgcagcgcagcgac

SEQ ID NO: 16462 - RNA, 5049 nt, Homo sapiens
  source 1..5049: mol_type = other RNA
gtcctaggaggctcctctgtggccaggcttctgcctccctgcaccctgagggaccattcgggtgcctcagggatgcccttccctcccaggggcactgacagcactggctgaaaggtctgaagagccagaggaggagccctgctggctggcccaggatggggcaaggagggagggaaagccaggggatggggagggacatgagatggagtttaaggcacacagcgagcgatggaggagggaggtgctggcctctcccctctgaattaactcccccaggagctcagctctggcctcagtttggtgaggttcagaagactcccagcaataaaaagtatttcttggatgatcaagtcctcccttactccagcctcctcttctcagctccccaggtggtgtgggaggggcccagtggcctggggtggggggtaaggggcgacgggatgacagagactgctgctgctctcaggcgggcaagggaggccctgatggcgccagtaccgcggggcagagcaccagctgcggggctgctaaggcgtcacctgcgtacctttccgggcctgctgaaaagctcacaccatcctccatgcatcagaaggggaagcggaaagtgaaaggatcctcccccgagtctactctgcattctgcccacccagctgcttgcccccattccagggcccctgcaggacaggccaccccaggaggcctccactcatttgagatttcagaagattcagggaccctggagcttagggagggggagcacccaccacttccttggtctgctgatgaggtctctgctgctctctccctggaggggagtgggtggaaggtcaagaggggagagatggaagtaaaagcagaaaacaaaaccaaaccagaaaaccaccggtttgtaaattggcaacaagacctgcctgctggctgccctgaggcccacgggtctgctcccacagaggaaggaggcaggaagcggctggcaggctccagctcccgcccggccccgctgagggctggccagcctcatggctccgaggccgggactcctgccatgcgcctaacaggtccaaggtcctctccggtctgggagctgccctctgcgcccctcgagcattctcctggatcccggcgtctgctcctaggtcttctcttcccggtctgtttttctccttgttatgttcctgggtttaattttcagagacagttcccatagggcctcctcagccaggtggtcactgaagtcattgaagaagtttataatgtcgtcgttcctccgcatgtcatagtgcgcctgctggaagcagcgcatgctgtcgaggatgttgaactgctgccaccgcttggagaagttcactttcccgtcgatgtagtctgggtttcccaggtgaacgaaggtcaggtcctgcaggatcagccccaggtacgggatgcacggcggttccacctccgagagggcggcccggtaggctcggaaggaggacgagctgtcgatcagtgtgcagtactcggccaggccctctgaagtctgcttctgccactccagcctgcggatgggcgccgagtccagggcagagaggatggccaagtaggagttgaagttattcagcttccgcaagtgcttcatgatcttgatgaacttcaagagcagccgttccctgtcctgggccttttcctgtaacatgattatggaccggacccagtaggacatgttgttgaagtgctccgtgaactgggtcaagttggggctcttctcctcattctgctcttttgcccaaagcaaaacctcaggaatctctattttatagaagagctcagcatccagcagcgttagctgctccgctatctcatggctgtgaaagtcgtgcaaggtccccggcctggctgctaccccccgggctgccaggggctggctggaggtggcacacctgagtagcttcttctggtccaccttgtccaggatgttcttccggagcacacgggccaggctcagctccccattgcacaccaggcggaagaccagttccatcagcagcttcaggatctcttctgtcaactccaccaggcagagctcatccaccacccgtaccagcacgaagaacgtgttcttgctgacgcgcttcttgaatgtgtcggcaaagggagagaatttctcatatctgtactgcagcttcttgatgagctcctctggggagatgaaggtcctgtaggtggtcaggaatgcctcgcagtacaacaccaaatctttcctgtcagtctcagtagcatggaccagtaagatgtccccagatcctccgcggacgtccggcccgtcatcaccctcctgcttgagcgtcagcctggacataatttcgttgtggtcaatgagggacagctcgtccacttcctcctccgactgagccgactccagagcatctggtgactttggggccctctcactgccgtctctgctgtccttcccagggacgccgctgaccgctgagggatctctgggatgtccgtctttcccagccggtggctctcctcgagagggagccagctcctcgctgctctggccagaggaatacagattgacatattcaccctcaccagcttcctcactggcgttttcactcgagtcagtgaaagaggtttcggaaggaaggcagacagtattcccatgaaagctgctctcctgagaagccgagagaggcccgtccacggtgctgggaggtggaccggccatggttggcacggctaagtcagagctctgagactggtgggcaggtgggaaatgtggagaggaagaggaggtaggcggaaggaaaggcggaacggaagcttggtggtgaggcacgaaatcctgggagtaggacctaaacacagacttatacgagggcacgggcaagctgccgtgccggctgagaaaggagttagagacggacacactgaggccctgagcggcactgccgtcctcgggggtgaaggccactttagtttgctggacacagtgggagacagaggagaaggaagaagcagcacaggaggcctgcagctgccgctgcttggggggtagggcgggcggcggggccagctcctgcacggagtccaccccactgaaggagtcgctgaagccgtatacctccatgaggagcttgttcttctgctggtagatgtgctcgttctgtggcgtctggtagaacatagagggctgcggctccgagtagtcctccagcaactgcatgtaggccagcatgtgtttgtttttcttctctggtagaggaggtggtttttctgggtcaccggttgactcaggagcagtaaaatcacccacaaattcgacaggggctgaggaacctccatgctgaaagggcagaatagcagcaaagggcgcgtaggggacggatgggatcggggctgtgctctgcaggtcctccccagagatgttgtcatactgcgagggatgccgctcgtaggacaccctgcagccagagccgtccgccgtctgggaggctgcgctcctgcgcttcttctcggggagagcaggtggcgtatctgtctgctgccctggggccagaggtccgtctggctggggatggccgccaagaggcagctggaaaggagggccaagaaatggagacccagactcccccaaagactctggcaacgggctaaggttccaggccgtctgctgaggtatctggtctgcgttagagaggtcttgctggaggaattcatagtcgggatcatagtggtctagtgtttcacagcttgtgttccgggagcactgcccactgtccctgtccagagaggacagctgctcgtctgacttgctgagcttgcctatgctgctgcagggggagaggcggggcgactctccaccatatgagtggctgcctcctgacagtcgcctctgtgcgtaacagtcaacatcaaaatcctgcctattgattccaacaggcaaactggagccactggtggctcggctcatgggggccaccacagccactcgggtaggggacggcgccgactgtcttttcttgggtggcaatgctggtggaggactattatcaaccacccgaatgccaggcagaggaggcttggggggcgcgacctcttcatccgtggcatctgggaggagctcagttgactgtgacatcccagtcgtcttgtttaggatctctacctcgcggtctgtcagggggagctctgctgggccatcaggcttgctggcaggggaactgggcttcacggggctcgtcggagacggacgtccctgcttctcgatggtgagcctgaccagctccttcactccatccagcacagccttgatgacccccttcacagtcgtcaccatctccttgtcttctgagttcacgccttccagcatcacttggtcagaccagcgaatgaggttggcgaggctttggtacactcggctatagcaggaagagagggctgagctgtgctgaattcgaggatcgttctgcaccaggggtaagatggcctccagcaccttgctggctgaccctggaagcatctccagtaccttcttatcaattgccattttgtccacaatggtcttaaagtagcgcagggcactgacaacttccttctctttctcctccagccagctcaggttcttctgcctttgagacctggaagccacagcactggtggacataaattctactgcctgctgctccagatccaaggggagagggtagccctctggtagaaatctgtctgttgcctcctggaagagaggaaacctggattctttgttcacaggcttctctggaatctttacggacacctcagctggttttcccttctttgatggcgttctcttgattttgggtgagtggaatttgtccatcagcttcatggtgaaggaagagagatgagaacgctgagagtctgccagagacgtgaagagaattcccagactcgctcctcttataaaccacagatgctgcttgaggggatggaagggacgcctctgagactcagagcggcttccctcccggagcccaatcaagtggttaaatcagcagcggctgtttttaaacttcc

SEQ ID NO: 16463 - RNA, 4994 nt, Homo sapiens
  source 1..4994: mol_type = other RNA
gtcctaggaggctcctctgtggccaggcttctgcctccctgcaccctgagggaccattcgggtgcctcagggatgcccttccctcccaggggcactgacagcactggctgaaaggtctgaagagccagaggaggagccctgctggctggcccaggatggggcaaggagggagggaaagccaggggatggggagggacatgagatggagtttaaggcacacagcgagcgatggaggagggaggtgctggcctctcccctctgaattaactcccccaggagctcagctctggcctcagtttggtgaggttcagaagactcccagcaataaaaagtatttcttggatgatcaagtcctcccttactccagcctcctcttctcagctccccaggtggtgtgggaggggcccagtggcctggggtggggggtaaggggcgacgggatgacagagactgctgctgctctcaggcgggcaagggaggccctgatggcgccagtaccgcggggcagagcaccagctgcggggctgctaaggcgtcacctgcgtacctttccgggcctgctgaaaagctcacaccatcctccatgcatcagaaggggaagcggaaagtgaaaggatcctcccccgagtctactctgcattctgcccacccagctgcttgcccccattccagggcccctgcaggacaggccaccccaggaggcctccactcatttgagatttcagaagattcagggaccctggagcttagggagggggagcacccaccacttccttggtctgctgatgaggtctctgctgctctctccctggaggggagtgggtggaaggtcaagaggggagagatggaagtaaaagcagaaaacaaaaccaaaccagaaaaccaccggtttgtaaattggcaacaagacctgcctgctggctgccctgaggcccacgggtctgctcccacagaggaaggaggcaggaagcggctggcaggctccagctcccgcccggccccgctgagggctggccagcctcatggctccgaggccgggactcctgccatgcgcctaacaggtccaaggtcctctccggtctgggagctgccctctgcgcccctcgagcattctcctggatcccggcgtctgctcctaggtcttctcttcccggtctgtttttctccttgttatgttcctgggtttaattttcagagacagttcccatagggcctcctcagccaggtggtcactgaagtcattgaagaagtttataatgtcgtcgttcctccgcatgtcatagtgcgcctgctggaagcagcgcatgctgtcgaggatgttgaactgctgccaccgcttggagaagttcactttcccgtcgatgtagtctgggtttcccaggtgaacgaaggtcaggtcctgcaggatcagccccaggtacgggatgcacggcggttccacctccgagagggcggcccggtaggctcggaaggaggacgagctgtcgatcagtgtgcagtactcggccaggccctctgaagtctgcttctgccactccagcctgcggatgggcgccgagtccagggcagagaggatggccaagtaggagttgaagttattcagcttccgcaagtgcttcatgatcttgatgaacttcaagagcagccgttccctgtcctgggccttttcctgtaacatgattatggaccggacccagtaggacatgttgttgaagtgctccgtgaactgggtcaagttggggctcttctcctcattctgctcttttgcccaaagcaaaacctcaggaatctctattttatagaagagctcagcatccagcagcgttagctgctccgctatctcatggctgtgaaagtcgtgcaaggtccccggcctggctgctaccccccgggctgccaggggctggctggaggtggcacacctgagtagcttcttctggtccaccttgtccaggatgttcttccggagcacacgggccaggctcagctccccattgcacaccaggcggaagaccagttccatcagcagcttcaggatctcttctgtcaactccaccaggcagagctcatccaccacccgtaccagcacgaagaacgtgttcttgctgacgcgcttcttgaatgtgtcggcaaagggagagaatttctcatatctgtactgcagcttcttgatgagctcctctggggagatgaaggtcctgtaggtggtcaggaatgcctcgcagtacaacaccaaatctttcctgtcagtctcagtagcatggaccagtaagatgtccccagatcctccgcggacgtccggcccgtcatcaccctcctgcttgagcgtcagcctggacataatttcgttgtggtcaatgagggacagctcgtccacttcctcctccgactgagccgactccagagcatctggtgactttggggccctctcactgccgtctctgctgtccttcccagggacgccgctgaccgctgagggatctctgggatgtccgtctttcccagccggtggctctcctcgagagggagccagctcctcgctgctctggccagaggaatacagattgacatattcaccctcaccagcttcctcactggcgttttcactcgagtcagtgaaagaggtttcggaaggaaggcagacagtattcccatgaaagctgctctcctgagaagccgagagaggcccgtccacggtgctgggaggtggaccggccatggttggcacggctaagtcagagctctgagactggtgggcaggtgggaaatgtggagaggaagaggaggtaggcggaaggaaaggcggaacggaagcttggtggtgaggcacgaaatcctgggagtaggacctaaacacagacttatacgagggcacgggcaagctgccgtgccggctgagaaaggagttagagacggacacactgaggccctgagcggcactgccgtcctcgggggtgaaggccactttagtttgctggacacagtgggagacagaggagaaggaagaagcagcacaggaggcctgcagctgccgctgcttggggggtagggcgggcggcggggccagctcctgcacggagtccaccccactgaaggagtcgctgaagccgtatacctccatgaggagcttgttcttctgctggtagatgtgctcgttctgtggcgtctggtagaacatagagggctgcggctccgagtagtcctccagcaactgcatgtaggccagcatgtgtttgtttttcttctctggtagaggaggtggtttttctgggtcaccggttgactcaggagcagtaaaatcacccacaaattcgacaggggctgaggaacctccatgctgaaagggcagaatagcagcaaagggcgcgtaggggacggatgggatcggggctgtgctctgcaggtcctccccagagatgttgtcatactgcgagggatgccgctcgtaggacaccctgcagccagagccgtccgccgtctgggaggctgcgctcctgcgcttcttctcggggagagcaggtggcgtatctgtctgctgccctggggccagaggtccgtctggctggggatggccgccaagaggcagctggaaaggagggccaagaaatggagacccagactcccccaaagactctggcaacgggctaaggttccaggccgtctgctgaggtatctggtctgcgttagagaggtcttgctggaggaattcatagtcgggatcatagtggtctagtgtttcacagcttgtgttccgggagcactgcccactgtccctgtccagagaggacagctgctcgtctgacttgctgagcttgcctatgctgctgcagggggagaggcggggcgactctccaccatatgagtggctgcctcctgacagtcgcctctgtgcgtaacagtcaacatcaaaatcctgcctattgattccaacaggcaaactggagccactggtggctcggctcatgggggccaccacagccactcgggtaggggacggcgccgactgtcttttcttgggtggcaatgctggtggaggactattatcaaccacccgaatgccaggcagaggaggcttggggggcgcgacctcttcatccgtggcatctgggaggagctcagttgactgtgacatcccagtcgtcttgtttaggatctctacctcgcggtctgtcagggggagctctgctgggccatcaggcttgctggcaggggaactgggcttcacggggctcgtcggagacggacgtccctgcttctcgatggtgagcctgaccagctccttcactccatccagcacagccttgatgacccccttcacagtcgtcaccatctccttgtcttctgagttcacgccttccagcatcacttggtcagaccagcgaatgaggttggcgaggctttggtacactcggctatagcaggaagagagggctgagctgtgctgaattcgaggatcgttctgcaccaggggtaagatggcctccagcaccttgctggctgaccctggaagcatctccagtaccttcttatcaattgccattttgtccacaatggtcttaaagtagcgcagggcactgacaacttccttctctttctcctccagccagctcaggttcttctgcctttgagacctggaagccacagcactggtggacataaattctactgcctgctgctccagatccaaggggagagggtagccctctggtagaaatctgtctgttgcctcctggaagagaggaaacctggattctttgttcacaggcttctctggaatctttacggacacctcagctggttttcccttctttgatggcgttctcttgattttgggtgagtggaatttgtccatcagcttcatggtgaaggaagagagatgagaacgctgagagtctgctttctcgatcttgccggacatttccgggctgcgccggaggccgaggccgccgctcatcgggcccgggccgggccgccgcggggcgacaggggcggcg

SEQ ID NO: 16464 - RNA, 4991 nt, Homo sapiens
  source 1..4991: mol_type = other RNA
gtcctaggaggctcctctgtggccaggcttctgcctccctgcaccctgagggaccattcgggtgcctcagggatgcccttccctcccaggggcactgacagcactggctgaaaggtctgaagagccagaggaggagccctgctggctggcccaggatggggcaaggagggagggaaagccaggggatggggagggacatgagatggagtttaaggcacacagcgagcgatggaggagggaggtgctggcctctcccctctgaattaactcccccaggagctcagctctggcctcagtttggtgaggttcagaagactcccagcaataaaaagtatttcttggatgatcaagtcctcccttactccagcctcctcttctcagctccccaggtggtgtgggaggggcccagtggcctggggtggggggtaaggggcgacgggatgacagagactgctgctgctctcaggcgggcaagggaggccctgatggcgccagtaccgcggggcagagcaccagctgcggggctgctaaggcgtcacctgcgtacctttccgggcctgctgaaaagctcacaccatcctccatgcatcagaaggggaagcggaaagtgaaaggatcctcccccgagtctactctgcattctgcccacccagctgcttgcccccattccagggcccctgcaggacaggccaccccaggaggcctccactcatttgagatttcagaagattcagggaccctggagcttagggagggggagcacccaccacttccttggtctgctgatgaggtctctgctgctctctccctggaggggagtgggtggaaggtcaagaggggagagatggaagtaaaagcagaaaacaaaaccaaaccagaaaaccaccggtttgtaaattggcaacaagacctgcctgctggctgccctgaggcccacgggtctgctcccacagaggaaggaggcaggaagcggctggcaggctccagctcccgcccggccccgctgagggctggccagcctcatggctccgaggccgggactcctgccatgcgcctaacaggtccaaggtcctctccggtctgggagctgccctctgcgcccctcgagcattctcctggatcccggcgtctgctcctaggtcttctcttcccggtctgtttttctccttgttatgttcctgggtttaattttcagagacagttcccatagggcctcctcagccaggtggtcactgaagtcattgaagaagtttataatgtcgtcgttcctccgcatgtcatagtgcgcctgctggaagcagcgcatgctgtcgaggatgttgaactgctgccaccgcttggagaagttcactttcccgtcgatgtagtctgggtttcccaggtgaacgaaggtcaggtcctgcaggatcagccccaggtacgggatgcacggcggttccacctccgagagggcggcccggtaggctcggaaggaggacgagctgtcgatcagtgtgcagtactcggccaggccctctgaagtctgcttctgccactccagcctgcggatgggcgccgagtccagggcagagaggatggccaagtaggagttgaagttattcagcttccgcaagtgcttcatgatcttgatgaacttcaagagcagccgttccctgtcctgggccttttcctgtaacatgattatggaccggacccagtaggacatgttgttgaagtgctccgtgaactgggtcaagttggggctcttctcctcattctgctcttttgcccaaagcaaaacctcaggaatctctattttatagaagagctcagcatccagcagcgttagctgctccgctatctcatggctgtgaaagtcgtgcaaggtccccggcctggctgctaccccccgggctgccaggggctggctggaggtggcacacctgagtagcttcttctggtccaccttgtccaggatgttcttccggagcacacgggccaggctcagctccccattgcacaccaggcggaagaccagttccatcagcagcttcaggatctcttctgtcaactccaccaggcagagctcatccaccacccgtaccagcacgaagaacgtgttcttgctgacgcgcttcttgaatgtgtcggcaaagggagagaatttctcatatctgtactgcagcttcttgatgagctcctctggggagatgaaggtcctgtaggtggtcaggaatgcctcgcagtacaacaccaaatctttcctgtcagtctcagtagcatggaccagtaagatgtccccagatcctccgcggacgtccggcccgtcatcaccctcctgcttgagcgtcagcctggacataatttcgttgtggtcaatgagggacagctcgtccacttcctcctccgactgagccgactccagagcatctggtgactttggggccctctcactgccgtctctgctgtccttcccagggacgccgctgaccgctgagggatctctgggatgtccgtctttcccagccggtggctctcctcgagagggagccagctcctcgctgctctggccagaggaatacagattgacatattcaccctcaccagcttcctcactggcgttttcactcgagtcagtgaaagaggtttcggaaggaaggcagacagtattcccatgaaagctgctctcctgagaagccgagagaggcccgtccacggtgctgggaggtggaccggccatggttggcacggctaagtcagagctctgagactggtgggcaggtgggaaatgtggagaggaagaggaggtaggcggaaggaaaggcggaacggaagcttggtggtgaggcacgaaatcctgggagtaggacctaaacacagacttatacgagggcacgggcaagctgccgtgccggctgagaaaggagttagagacggacacactgaggccctgagcggcactgccgtcctcgggggtgaaggccactttagtttgctggacacagtgggagacagaggagaaggaagaagcagcacaggaggcctgcagctgccgctgcttggggggtagggcgggcggcggggccagctcctgcacggagtccaccccactgaaggagtcgctgaagccgtatacctccatgaggagcttgttcttctgctggtagatgtgctcgttctgtggcgtctggtagaacatagagggctgcggctccgagtagtcctccagcaactgcatgtaggccagcatgtgtttgtttttcttctctggtagaggaggtggtttttctgggtcaccggttgactcaggagcagtaaaatcacccacaaattcgacaggggctgaggaacctccatgctgaaagggcagaatagcagcaaagggcgcgtaggggacggatgggatcggggctgtgctctgcaggtcctccccagagatgttgtcatactgcgagggatgccgctcgtaggacaccctgcagccagagccgtccgccgtctgggaggctgcgctcctgcgcttcttctcggggagagcaggtggcgtatctgtctgctgccctggggccagaggtccgtctggctggggatggccgccaagaggcagctggaaaggagggccaagaaatggagacccagactcccccaaagactctggcaacgggctaaggttccaggccgtctgctgaggtatctggtctgcgttagagaggtcttgctggaggaattcatagtcgggatcatagtggtctagtgtttcacagcttgtgttccgggagcactgcccactgtccctgtccagagaggacagctgctcgtctgacttgctgagcttgcctatgctgctgcagggggagaggcggggcgactctccaccatatgagtggctgcctcctgacagtcgcctctgtgcgtaacagtcaacatcaaaatcctgcctattgattccaacaggcaaactggagccactggtggctcggctcatgggggccaccacagccactcgggtaggggacggcgccgactgtcttttcttgggtggcaatgctggtggaggactattatcaaccacccgaatgccaggcagaggaggcttggggggcgcgacctcttcatccgtggcatctgggaggagctcagttgactgtgacatcccagtcgtcttgtttaggatctctacctcgcggtctgtcagggggagctctgctgggccatcaggcttgctggcaggggaactgggcttcacggggctcgtcggagacggacgtccctgcttctcgatggtgagcctgaccagctccttcactccatccagcacagccttgatgacccccttcacagtcgtcaccatctccttgtcttctgagttcacgccttccagcatcacttggtcagaccagcgaatgaggttggcgaggctttggtacactcggctatagcaggaagagagggctgagctgtgctgaattcgaggatcgttctgcaccaggggtaagatggcctccagcaccttgctggctgaccctggaagcatctccagtaccttcttatcaattgccattttgtccacaatggtcttaaagtagcgcagggcactgacaacttccttctctttctcctccagccagctcaggttcttctgcctttgagacctggaagccacagcactggtggacataaattctactgcctgctgctccagatccaaggggagagggtagccctctggtagaaatctgtctgttgcctcctggaagagaggaaacctggattctttgttcacaggcttctctggaatctttacggacacctcagctggttttcccttctttgatggcgttctcttgattttgggtgagtggaatttgtccatcagcttcatggtgaaggaagagagatgagaacgctgagagtctggaacagctcaacagggtcaggaggctctcaacaccagccctcatatgtcagcagtcatccctcgcattcaaatgaactgggatggtgtgacttct

SEQ ID NO: 16465 - RNA, 5256 nt, Homo sapiens
  source 1..5256: mol_type = other RNA
gtcctaggaggctcctctgtggccaggcttctgcctccctgcaccctgagggaccattcgggtgcctcagggatgcccttccctcccaggggcactgacagcactggctgaaaggtctgaagagccagaggaggagccctgctggctggcccaggatggggcaaggagggagggaaagccaggggatggggagggacatgagatggagtttaaggcacacagcgagcgatggaggagggaggtgctggcctctcccctctgaattaactcccccaggagctcagctctggcctcagtttggtgaggttcagaagactcccagcaataaaaagtatttcttggatgatcaagtcctcccttactccagcctcctcttctcagctccccaggtggtgtgggaggggcccagtggcctggggtggggggtaaggggcgacgggatgacagagactgctgctgctctcaggcgggcaagggaggccctgatggcgccagtaccgcggggcagagcaccagctgcggggctgctaaggcgtcacctgcgtacctttccgggcctgctgaaaagctcacaccatcctccatgcatcagaaggggaagcggaaagtgaaaggatcctcccccgagtctactctgcattctgcccacccagctgcttgcccccattccagggcccctgcaggacaggccaccccaggaggcctccactcatttgagatttcagaagattcagggaccctggagcttagggagggggagcacccaccacttccttggtctgctgatgaggtctctgctgctctctccctggaggggagtgggtggaaggtcaagaggggagagatggaagtaaaagcagaaaacaaaaccaaaccagaaaaccaccggtttgtaaattggcaacaagacctgcctgctggctgccctgaggcccacgggtctgctcccacagaggaaggaggcaggaagcggctggcaggctccagctcccgcccggccccgctgagggctggccagcctcatggctccgaggccgggactcctgccatgcgcctaacaggtccaaggtcctctccggtctgggagctgccctctgcgcccctcgagcattctcctggatcccggcgtctgctcctaggtcttctcttcccggtctgtttttctccttgttatgttcctgggtttaattttcagagacagttcccatagggcctcctcagccaggtggtcactgaagtcattgaagaagtttataatgtcgtcgttcctccgcatgtcatagtgcgcctgctggaagcagcgcatgctgtcgaggatgttgaactgctgccaccgcttggagaagttcactttcccgtcgatgtagtctgggtttcccaggtgaacgaaggtcaggtcctgcaggatcagccccaggtacgggatgcacggcggttccacctccgagagggcggcccggtaggctcggaaggaggacgagctgtcgatcagtgtgcagtactcggccaggccctctgaagtctgcttctgccactccagcctgcggatgggcgccgagtccagggcagagaggatggccaagtaggagttgaagttattcagcttccgcaagtgcttcatgatcttgatgaacttcaagagcagccgttccctgtcctgggccttttcctgtaacatgattatggaccggacccagtaggacatgttgttgaagtgctccgtgaactgggtcaagttggggctcttctcctcattctgctcttttgcccaaagcaaaacctcaggaatctctattttatagaagagctcagcatccagcagcgttagctgctccgctatctcatggctgtgaaagtcgtgcaaggtccccggcctggctgctaccccccgggctgccaggggctggctggaggtggcacacctgagtagcttcttctggtccaccttgtccaggatgttcttccggagcacacgggccaggctcagctccccattgcacaccaggcggaagaccagttccatcagcagcttcaggatctcttctgtcaactccaccaggcagagctcatccaccacccgtaccagcacgaagaacgtgttcttgctgacgcgcttcttgaatgtgtcggcaaagggagagaatttctcatatctgtactgcagcttcttgatgagctcctctggggagatgaaggtcctgtaggtggtcaggaatgcctcgcagtacaacaccaaatctttcctgtcagtctcagtagcatggaccagtaagatgtccccagatcctccgcggacgtccggcccgtcatcaccctcctgcttgagcgtcagcctggacataatttcgttgtggtcaatgagggacagctcgtccacttcctcctccgactgagccgactccagagcatctggtgactttggggccctctcactgccgtctctgctgtccttcccagggacgccgctgaccgctgagggatctctgggatgtccgtctttcccagccggtggctctcctcgagagggagccagctcctcgctgctctggccagaggaatacagattgacatattcaccctcaccagcttcctcactggcgttttcactcgagtcagtgaaagaggtttcggaaggaaggcagacagtattcccatgaaagctgctctcctgagaagccgagagaggcccgtccacggtgctgggaggtggaccggccatggttggcacggctaagtcagagctctgagactggtgggcaggtgggaaatgtggagaggaagaggaggtaggcggaaggaaaggcggaacggaagcttggtggtgaggcacgaaatcctgggagtaggacctaaacacagacttatacgagggcacgggcaagctgccgtgccggctgagaaaggagttagagacggacacactgaggccctgagcggcactgccgtcctcgggggtgaaggccactttagtttgctggacacagtgggagacagaggagaaggaagaagcagcacaggaggcctgcagctgccgctgcttggggggtagggcgggcggcggggccagctcctgcacggagtccaccccactgaaggagtcgctgaagccgtatacctccatgaggagcttgttcttctgctggtagatgtgctcgttctgtggcgtctggtagaacatagagggctgcggctccgagtagtcctccagcaactgcatgtaggccagcatgtgtttgtttttcttctctggtagaggaggtggtttttctgggtcaccggttgactcaggagcagtaaaatcacccacaaattcgacaggggctgaggaacctccatgctgaaagggcagaatagcagcaaagggcgcgtaggggacggatgggatcggggctgtgctctgcaggtcctccccagagatgttgtcatactgcgagggatgccgctcgtaggacaccctgcagccagagccgtccgccgtctgggaggctgcgctcctgcgcttcttctcggggagagcaggtggcgtatctgtctgctgccctggggccagaggtccgtctggctggggatggccgccaagaggcagctggaaaggagggccaagaaatggagacccagactcccccaaagactctggcaacgggctaaggttccaggccgtctgctgaggtatctggtctgcgttagagaggtcttgctggaggaattcatagtcgggatcatagtggtctagtgtttcacagcttgtgttccgggagcactgcccactgtccctgtccagagaggacagctgctcgtctgacttgctgagcttgcctatgctgctgcagggggagaggcggggcgactctccaccatatgagtggctgcctcctgacagtcgcctctgtgcgtaacagtcaacatcaaaatcctgcctattgattccaacaggcaaactggagccactggtggctcggctcatgggggccaccacagccactcgggtaggggacggcgccgactgtcttttcttgggtggcaatgctggtggaggactattatcaaccacccgaatgccaggcagaggaggcttggggggcgcgacctcttcatccgtggcatctgggaggagctcagttgactgtgacatcccagtcgtcttgtttaggatctctacctcgcggtctgtcagggggagctctgctgggccatcaggcttgctggcaggggaactgggcttcacggggctcgtcggagacggacgtccctgcttctcgatggtgagcctgaccagctccttcactccatccagcacagccttgatgacccccttcacagtcgtcaccatctccttgtcttctgagttcacgccttccagcatcacttggtcagaccagcgaatgaggttggcgaggctttggtacactcggctatagcaggaagagagggctgagctgtgctgaattcgaggatcgttctgcaccaggggtaagatggcctccagcaccttgctggctgaccctggaagcatctccagtaccttcttatcaattgccattttgtccacaatggtcttaaagtagcgcagggcactgacaacttccttctctttctcctccagccagctcaggttcttctgcctttgagacctggaagccacagcactggtggacataaattctactgcctgctgctccagatccaaggggagagggtagccctctggtagaaatctgtctgttgcctcctggaagagaggaaacctggattctttgttcacaggcttctctggaatctttacggacacctcagctggttttcccttctttgatggcgttctcttgattttgggtgagtggaatttgtccatcagcttcatggtgaaggaagagagatgagaacgctgagagtctggaacgacacctcctgtcctcttgttctgttccaaggttgtcaggctgggacgaaatcccaagaaagaaatgggcatgtggtcactatcatagcagactgccagttagggacatcagaatatatttctctgtcctcaagttaggaagtgagaggacaaacctggccttctgtgttgtttcagccactaattggttttgtcaattaggcaaaacataatttctctaagcctcttttctcatccacaggcattagcctagtcagcggttctcaaagtgtggtcctgaaccaacaacgacggcagcttcaccaagagacttcttagaaatgcaaattcttgggcccatgccacacctacagaag

SEQ ID NO: 16466 - RNA, 5125 nt, Homo sapiens
  source 1..5125: mol_type = other RNA
gtcctaggaggctcctctgtggccaggcttctgcctccctgcaccctgagggaccattcgggtgcctcagggatgcccttccctcccaggggcactgacagcactggctgaaaggtctgaagagccagaggaggagccctgctggctggcccaggatggggcaaggagggagggaaagccaggggatggggagggacatgagatggagtttaaggcacacagcgagcgatggaggagggaggtgctggcctctcccctctgaattaactcccccaggagctcagctctggcctcagtttggtgaggttcagaagactcccagcaataaaaagtatttcttggatgatcaagtcctcccttactccagcctcctcttctcagctccccaggtggtgtgggaggggcccagtggcctggggtggggggtaaggggcgacgggatgacagagactgctgctgctctcaggcgggcaagggaggccctgatggcgccagtaccgcggggcagagcaccagctgcggggctgctaaggcgtcacctgcgtacctttccgggcctgctgaaaagctcacaccatcctccatgcatcagaaggggaagcggaaagtgaaaggatcctcccccgagtctactctgcattctgcccacccagctgcttgcccccattccagggcccctgcaggacaggccaccccaggaggcctccactcatttgagatttcagaagattcagggaccctggagcttagggagggggagcacccaccacttccttggtctgctgatgaggtctctgctgctctctccctggaggggagtgggtggaaggtcaagaggggagagatggaagtaaaagcagaaaacaaaaccaaaccagaaaaccaccggtttgtaaattggcaacaagacctgcctgctggctgccctgaggcccacgggtctgctcccacagaggaaggaggcaggaagcggctggcaggctccagctcccgcccggccccgctgagggctggccagcctcatggctccgaggccgggactcctgccatgcgcctaacaggtccaaggtcctctccggtctgggagctgccctctgcgcccctcgagcattctcctggatcccggcgtctgctcctaggtcttctcttcccggtctgtttttctccttgttatgttcctgggtttaattttcagagacagttcccatagggcctcctcagccaggtggtcactgaagtcattgaagaagtttataatgtcgtcgttcctccgcatgtcatagtgcgcctgctggaagcagcgcatgctgtcgaggatgttgaactgctgccaccgcttggagaagttcactttcccgtcgatgtagtctgggtttcccaggtgaacgaaggtcaggtcctgcaggatcagccccaggtacgggatgcacggcggttccacctccgagagggcggcccggtaggctcggaaggaggacgagctgtcgatcagtgtgcagtactcggccaggccctctgaagtctgcttctgccactccagcctgcggatgggcgccgagtccagggcagagaggatggccaagtaggagttgaagttattcagcttccgcaagtgcttcatgatcttgatgaacttcaagagcagccgttccctgtcctgggccttttcctgtaacatgattatggaccggacccagtaggacatgttgttgaagtgctccgtgaactgggtcaagttggggctcttctcctcattctgctcttttgcccaaagcaaaacctcaggaatctctattttatagaagagctcagcatccagcagcgttagctgctccgctatctcatggctgtgaaagtcgtgcaaggtccccggcctggctgctaccccccgggctgccaggggctggctggaggtggcacacctgagtagcttcttctggtccaccttgtccaggatgttcttccggagcacacgggccaggctcagctccccattgcacaccaggcggaagaccagttccatcagcagcttcaggatctcttctgtcaactccaccaggcagagctcatccaccacccgtaccagcacgaagaacgtgttcttgctgacgcgcttcttgaatgtgtcggcaaagggagagaatttctcatatctgtactgcagcttcttgatgagctcctctggggagatgaaggtcctgtaggtggtcaggaatgcctcgcagtacaacaccaaatctttcctgtcagtctcagtagcatggaccagtaagatgtccccagatcctccgcggacgtccggcccgtcatcaccctcctgcttgagcgtcagcctggacataatttcgttgtggtcaatgagggacagctcgtccacttcctcctccgactgagccgactccagagcatctggtgactttggggccctctcactgccgtctctgctgtccttcccagggacgccgctgaccgctgagggatctctgggatgtccgtctttcccagccggtggctctcctcgagagggagccagctcctcgctgctctggccagaggaatacagattgacatattcaccctcaccagcttcctcactggcgttttcactcgagtcagtgaaagaggtttcggaaggaaggcagacagtattcccatgaaagctgctctcctgagaagccgagagaggcccgtccacggtgctgggaggtggaccggccatggttggcacggctaagtcagagctctgagactggtgggcaggtgggaaatgtggagaggaagaggaggtaggcggaaggaaaggcggaacggaagcttggtggtgaggcacgaaatcctgggagtaggacctaaacacagacttatacgagggcacgggcaagctgccgtgccggctgagaaaggagttagagacggacacactgaggccctgagcggcactgccgtcctcgggggtgaaggccactttagtttgctggacacagtgggagacagaggagaaggaagaagcagcacaggaggcctgcagctgccgctgcttggggggtagggcgggcggcggggccagctcctgcacggagtccaccccactgaaggagtcgctgaagccgtatacctccatgaggagcttgttcttctgctggtagatgtgctcgttctgtggcgtctggtagaacatagagggctgcggctccgagtagtcctccagcaactgcatgtaggccagcatgtgtttgtttttcttctctggtagaggaggtggtttttctgggtcaccggttgactcaggagcagtaaaatcacccacaaattcgacaggggctgaggaacctccatgctgaaagggcagaatagcagcaaagggcgcgtaggggacggatgggatcggggctgtgctctgcaggtcctccccagagatgttgtcatactgcgagggatgccgctcgtaggacaccctgcagccagagccgtccgccgtctgggaggctgcgctcctgcgcttcttctcggggagagcaggtggcgtatctgtctgctgccctggggccagaggtccgtctggctggggatggccgccaagaggcagctggaaaggagggccaagaaatggagacccagactcccccaaagactctggcaacgggctaaggttccaggccgtctgctgaggtatctggtctgcgttagagaggtcttgctggaggaattcatagtcgggatcatagtggtctagtgtttcacagcttgtgttccgggagcactgcccactgtccctgtccagagaggacagctgctcgtctgacttgctgagcttgcctatgctgctgcagggggagaggcggggcgactctccaccatatgagtggctgcctcctgacagtcgcctctgtgcgtaacagtcaacatcaaaatcctgcctattgattccaacaggcaaactggagccactggtggctcggctcatgggggccaccacagccactcgggtaggggacggcgccgactgtcttttcttgggtggcaatgctggtggaggactattatcaaccacccgaatgccaggcagaggaggcttggggggcgcgacctcttcatccgtggcatctgggaggagctcagttgactgtgacatcccagtcgtcttgtttaggatctctacctcgcggtctgtcagggggagctctgctgggccatcaggcttgctggcaggggaactgggcttcacggggctcgtcggagacggacgtccctgcttctcgatggtgagcctgaccagctccttcactccatccagcacagccttgatgacccccttcacagtcgtcaccatctccttgtcttctgagttcacgccttccagcatcacttggtcagaccagcgaatgaggttggcgaggctttggtacactcggctatagcaggaagagagggctgagctgtgctgaattcgaggatcgttctgcaccaggggtaagatggcctccagcaccttgctggctgaccctggaagcatctccagtaccttcttatcaattgccattttgtccacaatggtcttaaagtagcgcagggcactgacaacttccttctctttctcctccagccagctcaggttcttctgcctttgagacctggaagccacagcactggtggacataaattctactgcctgctgctccagatccaaggggagagggtagccctctggtagaaatctgtctgttgcctcctggaagagaggaaacctggattctttgttcacaggcttctctggaatctttacggacacctcagctggttttcccttctttgatggcgttctcttgattttgggtgagtggaatttgtccatcagcttcatggtgaaggaagagagatgagaacgctgagagtctgtgtccatggcagcacggtcgctcggtctggcagcctgggtagcttagaaactgtgctaggttagacaagcttctctgggagcaggcactttcatctacaaccccctagcagaaggcggtgcccagaaaaggcccaaggacaaactatgctgaaatgaactggcctcaggtctttctcccaaatagcagagaactcaaatgaagagtcatttcattcccagcggtttggg

SEQ ID NO: 16467 - RNA, 5815 nt, Homo sapiens
  source 1..5815: mol_type = other RNA
gtcctaggaggctcctctgtggccaggcttctgcctccctgcaccctgagggaccattcgggtgcctcagggatgcccttccctcccaggggcactgacagcactggctgaaaggtctgaagagccagaggaggagccctgctggctggcccaggatggggcaaggagggagggaaagccaggggatggggagggacatgagatggagtttaaggcacacagcgagcgatggaggagggaggtgctggcctctcccctctgaattaactcccccaggagctcagctctggcctcagtttggtgaggttcagaagactcccagcaataaaaagtatttcttggatgatcaagtcctcccttactccagcctcctcttctcagctccccaggtggtgtgggaggggcccagtggcctggggtggggggtaaggggcgacgggatgacagagactgctgctgctctcaggcgggcaagggaggccctgatggcgccagtaccgcggggcagagcaccagctgcggggctgctaaggcgtcacctgcgtacctttccgggcctgctgaaaagctcacaccatcctccatgcatcagaaggggaagcggaaagtgaaaggatcctcccccgagtctactctgcattctgcccacccagctgcttgcccccattccagggcccctgcaggacaggccaccccaggaggcctccactcatttgagatttcagaagattcagggaccctggagcttagggagggggagcacccaccacttccttggtctgctgatgaggtctctgctgctctctccctggaggggagtgggtggaaggtcaagaggggagagatggaagtaaaagcagaaaacaaaaccaaaccagaaaaccaccggtttgtaaattggcaacaagacctgcctgctggctgccctgaggcccacgggtctgctcccacagaggaaggaggcaggaagcggctggcaggctccagctcccgcccggccccgctgagggctggccagcctcatggctccgaggccgggactcctgccatgcgcctaacaggtccaaggtcctctccggtctgggagctgccctctgcgcccctcgagcattctcctggatcccggcgtctgctcctaggtcttctcttcccggtctgtttttctccttgttatgttcctgggtttaattttcagagacagttcccatagggcctcctcagccaggtggtcactgaagtcattgaagaagtttataatgtcgtcgttcctccgcatgtcatagtgcgcctgctggaagcagcgcatgctgtcgaggatgttgaactgctgccaccgcttggagaagttcactttcccgtcgatgtagtctgggtttcccaggtgaacgaaggtcaggtcctgcaggatcagccccaggtacgggatgcacggcggttccacctccgagagggcggcccggtaggctcggaaggaggacgagctgtcgatcagtgtgcagtactcggccaggccctctgaagtctgcttctgccactccagcctgcggatgggcgccgagtccagggcagagaggatggccaagtaggagttgaagttattcagcttccgcaagtgcttcatgatcttgatgaacttcaagagcagccgttccctgtcctgggccttttcctgtaacatgattatggaccggacccagtaggacatgttgttgaagtgctccgtgaactgggtcaagttggggctcttctcctcattctgctcttttgcccaaagcaaaacctcaggaatctctattttatagaagagctcagcatccagcagcgttagctgctccgctatctcatggctgtgaaagtcgtgcaaggtccccggcctggctgctaccccccgggctgccaggggctggctggaggtggcacacctgagtagcttcttctggtccaccttgtccaggatgttcttccggagcacacgggccaggctcagctccccattgcacaccaggcggaagaccagttccatcagcagcttcaggatctcttctgtcaactccaccaggcagagctcatccaccacccgtaccagcacgaagaacgtgttcttgctgacgcgcttcttgaatgtgtcggcaaagggagagaatttctcatatctgtactgcagcttcttgatgagctcctctggggagatgaaggtcctgtaggtggtcaggaatgcctcgcagtacaacaccaaatctttcctgtcagtctcagtagcatggaccagtaagatgtccccagatcctccgcggacgtccggcccgtcatcaccctcctgcttgagcgtcagcctggacataatttcgttgtggtcaatgagggacagctcgtccacttcctcctccgactgagccgactccagagcatctggtgactttggggccctctcactgccgtctctgctgtccttcccagggacgccgctgaccgctgagggatctctgggatgtccgtctttcccagccggtggctctcctcgagagggagccagctcctcgctgctctggccagaggaatacagattgacatattcaccctcaccagcttcctcactggcgttttcactcgagtcagtgaaagaggtttcggaaggaaggcagacagtattcccatgaaagctgctctcctgagaagccgagagaggcccgtccacggtgctgggaggtggaccggccatggttggcacggctaagtcagagctctgagactggtgggcaggtgggaaatgtggagaggaagaggaggtaggcggaaggaaaggcggaacggaagcttggtggtgaggcacgaaatcctgggagtaggacctaaacacagacttatacgagggcacgggcaagctgccgtgccggctgagaaaggagttagagacggacacactgaggccctgagcggcactgccgtcctcgggggtgaaggccactttagtttgctggacacagtgggagacagaggagaaggaagaagcagcacaggaggcctgcagctgccgctgcttggggggtagggcgggcggcggggccagctcctgcacggagtccaccccactgaaggagtcgctgaagccgtatacctccatgaggagcttgttcttctgctggtagatgtgctcgttctgtggcgtctggtagaacatagagggctgcggctccgagtagtcctccagcaactgcatgtaggccagcatgtgtttgtttttcttctctggtagaggaggtggtttttctgggtcaccggttgactcaggagcagtaaaatcacccacaaattcgacaggggctgaggaacctccatgctgaaagggcagaatagcagcaaagggcgcgtaggggacggatgggatcggggctgtgctctgcaggtcctccccagagatgttgtcatactgcgagggatgccgctcgtaggacaccctgcagccagagccgtccgccgtctgggaggctgcgctcctgcgcttcttctcggggagagcaggtggcgtatctgtctgctgccctggggccagaggtccgtctggctggggatggccgccaagaggcagctggaaaggagggccaagaaatggagacccagactcccccaaagactctggcaacgggctaaggttccaggccgtctgctgaggtatctggtctgcgttagagaggtcttgctggaggaattcatagtcgggatcatagtggtctagtgtttcacagcttgtgttccgggagcactgcccactgtccctgtccagagaggacagctgctcgtctgacttgctgagcttgcctatgctgctgcagggggagaggcggggcgactctccaccatatgagtggctgcctcctgacagtcgcctctgtgcgtaacagtcaacatcaaaatcctgcctattgattccaacaggcaaactggagccactggtggctcggctcatgggggccaccacagccactcgggtaggggacggcgccgactgtcttttcttgggtggcaatgctggtggaggactattatcaaccacccgaatgccaggcagaggaggcttggggggcgcgacctcttcatccgtggcatctgggaggagctcagttgactgtgacatcccagtcgtcttgtttaggatctctacctcgcggtctgtcagggggagctctgctgggccatcaggcttgctggcaggggaactgggcttcacggggctcgtcggagacggacgtccctgcttctcgatggtgagcctgaccagctccttcactccatccagcacagccttgatgacccccttcacagtcgtcaccatctccttgtcttctgagttcacgccttccagcatcacttggtcagaccagcgaatgaggttggcgaggctttggtacactcggctatagcaggaagagagggctgagctgtgctgaattcgaggatcgttctgcaccaggggtaagatggcctccagcaccttgctggctgaccctggaagcatctccagtaccttcttatcaattgccattttgtccacaatggtcttaaagtagcgcagggcactgacaacttccttctctttctcctccagccagctcaggttcttctgcctttgagacctggaagccacagcactggtggacataaattctactgcctgctgctccagatccaaggggagagggtagccctctggtagaaatctgtctgttgcctcctggaagagaggaaacctggattctttgttcacaggcttctctggaatctttacggacacctcagctggttttcccttctttgatggcgttctcttgattttgggtgagtggaatttgtccatcagcttcatggtgaaggaagagagatgagaacgctgagagtcttgtttccaggggtacagatgacttcgtttcaagggcttctgtttttcaatagcattgcccattttaaagccagaggacacagggcccttcccagccccagcgtctttccggagcagcaactgaggaccgagtcactggctgaaaggggatatctcttggacatcccaaaccacccagcggcagaacccaggcagcctcacaagggaagcctgaggaatctcattctcaagtctttgccttctgcctttcaaaatccctttggccccagggaggaaatcagaagaaagggcttgttatcgccctaccggtgcctctcaggcatggtctatattaagaagctctttcctcagcatccttttgacactttattactcatcagcacaacagcggcttgcaagatgaattttatgtccaaatacttttaataccacttttctccgcaggagaaatggggaatcaggtgatcaaaatgctgaaagtcataaatgaaccattctggggcatgccaggagaaacattttcatacagacccttatgccacgccttctatttcagagtcccacgctcagaccagtgtgcaccacgtaacaagtactgtcagagaaaacaagctgatttcactaatgctgtgtttccaagggaaacacaaaacgaaacaaaacatcaaaacactgctacacctcagtctccaaagaagaaaacaccttggggacaaatacagctaagaatttataaccccaagctccaaactcccactgcactttgggaacaattttgctggagaaagtgctacgctacctaaattctgaacaaagggttttctagaagaaaagaagggaatgaaatcaatcacatattcttggtaaaaaggaagacaatgtcgaggtggatgaaaagatttcatttatttcagtcccaga

SEQ ID NO: 16468 - RNA, 5017 nt, Homo sapiens
  source 1..5017: mol_type = other RNA
gtcctaggaggctcctctgtggccaggcttctgcctccctgcaccctgagggaccattcgggtgcctcagggatgcccttccctcccaggggcactgacagcactggctgaaaggtctgaagagccagaggaggagccctgctggctggcccaggatggggcaaggagggagggaaagccaggggatggggagggacatgagatggagtttaaggcacacagcgagcgatggaggagggaggtgctggcctctcccctctgaattaactcccccaggagctcagctctggcctcagtttggtgaggttcagaagactcccagcaataaaaagtatttcttggatgatcaagtcctcccttactccagcctcctcttctcagctccccaggtggtgtgggaggggcccagtggcctggggtggggggtaaggggcgacgggatgacagagactgctgctgctctcaggcgggcaagggaggccctgatggcgccagtaccgcggggcagagcaccagctgcggggctgctaaggcgtcacctgcgtacctttccgggcctgctgaaaagctcacaccatcctccatgcatcagaaggggaagcggaaagtgaaaggatcctcccccgagtctactctgcattctgcccacccagctgcttgcccccattccagggcccctgcaggacaggccaccccaggaggcctccactcatttgagatttcagaagattcagggaccctggagcttagggagggggagcacccaccacttccttggtctgctgatgaggtctctgctgctctctccctggaggggagtgggtggaaggtcaagaggggagagatggaagtaaaagcagaaaacaaaaccaaaccagaaaaccaccggtttgtaaattggcaacaagacctgcctgctggctgccctgaggcccacgggtctgctcccacagaggaaggaggcaggaagcggctggcaggctccagctcccgcccggccccgctgagggctggccagcctcatggctccgaggccgggactcctgccatgcgcctaacaggtccaaggtcctctccggtctgggagctgccctctgcgcccctcgagcattctcctggatcccggcgtctgctcctaggtcttctcttcccggtctgtttttctccttgttatgttcctgggtttaattttcagagacagttcccatagggcctcctcagccaggtggtcactgaagtcattgaagaagtttataatgtcgtcgttcctccgcatgtcatagtgcgcctgctggaagcagcgcatgctgtcgaggatgttgaactgctgccaccgcttggagaagttcactttcccgtcgatgtagtctgggtttcccaggtgaacgaaggtcaggtcctgcaggatcagccccaggtacgggatgcacggcggttccacctccgagagggcggcccggtaggctcggaaggaggacgagctgtcgatcagtgtgcagtactcggccaggccctctgaagtctgcttctgccactccagcctgcggatgggcgccgagtccagggcagagaggatggccaagtaggagttgaagttattcagcttccgcaagtgcttcatgatcttgatgaacttcaagagcagccgttccctgtcctgggccttttcctgtaacatgattatggaccggacccagtaggacatgttgttgaagtgctccgtgaactgggtcaagttggggctcttctcctcattctgctcttttgcccaaagcaaaacctcaggaatctctattttatagaagagctcagcatccagcagcgttagctgctccgctatctcatggctgtgaaagtcgtgcaaggtccccggcctggctgctaccccccgggctgccaggggctggctggaggtggcacacctgagtagcttcttctggtccaccttgtccaggatgttcttccggagcacacgggccaggctcagctccccattgcacaccaggcggaagaccagttccatcagcagcttcaggatctcttctgtcaactccaccaggcagagctcatccaccacccgtaccagcacgaagaacgtgttcttgctgacgcgcttcttgaatgtgtcggcaaagggagagaatttctcatatctgtactgcagcttcttgatgagctcctctggggagatgaaggtcctgtaggtggtcaggaatgcctcgcagtacaacaccaaatctttcctgtcagtctcagtagcatggaccagtaagatgtccccagatcctccgcggacgtccggcccgtcatcaccctcctgcttgagcgtcagcctggacataatttcgttgtggtcaatgagggacagctcgtccacttcctcctccgactgagccgactccagagcatctggtgactttggggccctctcactgccgtctctgctgtccttcccagggacgccgctgaccgctgagggatctctgggatgtccgtctttcccagccggtggctctcctcgagagggagccagctcctcgctgctctggccagaggaatacagattgacatattcaccctcaccagcttcctcactggcgttttcactcgagtcagtgaaagaggtttcggaaggaaggcagacagtattcccatgaaagctgctctcctgagaagccgagagaggcccgtccacggtgctgggaggtggaccggccatggttggcacggctaagtcagagctctgagactggtgggcaggtgggaaatgtggagaggaagaggaggtaggcggaaggaaaggcggaacggaagcttggtggtgaggcacgaaatcctgggagtaggacctaaacacagacttatacgagggcacgggcaagctgccgtgccggctgagaaaggagttagagacggacacactgaggccctgagcggcactgccgtcctcgggggtgaaggccactttagtttgctggacacagtgggagacagaggagaaggaagaagcagcacaggaggcctgcagctgccgctgcttggggggtagggcgggcggcggggccagctcctgcacggagtccaccccactgaaggagtcgctgaagccgtatacctccatgaggagcttgttcttctgctggtagatgtgctcgttctgtggcgtctggtagaacatagagggctgcggctccgagtagtcctccagcaactgcatgtaggccagcatgtgtttgtttttcttctctggtagaggaggtggtttttctgggtcaccggttgactcaggagcagtaaaatcacccacaaattcgacaggggctgaggaacctccatgctgaaagggcagaatagcagcaaagggcgcgtaggggacggatgggatcggggctgtgctctgcaggtcctccccagagatgttgtcatactgcgagggatgccgctcgtaggacaccctgcagccagagccgtccgccgtctgggaggctgcgctcctgcgcttcttctcggggagagcaggtggcgtatctgtctgctgccctggggccagaggtccgtctggctggggatggccgccaagaggcagctggaaaggagggccaagaaatggagacccagactcccccaaagactctggcaacgggctaaggttccaggccgtctgctgaggtatctggtctgcgttagagaggtcttgctggaggaattcatagtcgggatcatagtggtctagtgtttcacagcttgtgttccgggagcactgcccactgtccctgtccagagaggacagctgctcgtctgacttgctgagcttgcctatgctgctgcagggggagaggcggggcgactctccaccatatgagtggctgcctcctgacagtcgcctctgtgcgtaacagtcaacatcaaaatcctgcctattgattccaacaggcaaactggagccactggtggctcggctcatgggggccaccacagccactcgggtaggggacggcgccgactgtcttttcttgggtggcaatgctggtggaggactattatcaaccacccgaatgccaggcagaggaggcttggggggcgcgacctcttcatccgtggcatctgggaggagctcagttgactgtgacatcccagtcgtcttgtttaggatctctacctcgcggtctgtcagggggagctctgctgggccatcaggcttgctggcaggggaactgggcttcacggggctcgtcggagacggacgtccctgcttctcgatggtgagcctgaccagctccttcactccatccagcacagccttgatgacccccttcacagtcgtcaccatctccttgtcttctgagttcacgccttccagcatcacttggtcagaccagcgaatgaggttggcgaggctttggtacactcggctatagcaggaagagagggctgagctgtgctgaattcgaggatcgttctgcaccaggggtaagatggcctccagcaccttgctggctgaccctggaagcatctccagtaccttcttatcaattgccattttgtccacaatggtcttaaagtagcgcagggcactgacaacttccttctctttctcctccagccagctcaggttcttctgcctttgagacctggaagccacagcactggtggacataaattctactgcctgctgctccagatccaaggggagagggtagccctctggtagaaatctgtctgttgcctctttgttcacaggcttctctggaatctttacggacacctcagctggttttcccttctttgatggcgttctcttgattttgggtgagtggaatttgtccatcagcttcatggtgaaggaagagagatgagaacgctgagagtctgccagagacgtgaagagaattcccagactcgctcctcttataaaccacagatgctgcttgaggggatggaagggacgcctctgagactcagagcggcttccctcccggagcccaatcaagtggttaaatcagcagcggctgttttt

SEQ ID NO: 16469 - RNA, 5168 nt, Homo sapiens
  source 1..5168: mol_type = other RNA
gtcctaggaggctcctctgtggccaggcttctgcctccctgcaccctgagggaccattcgggtgcctcagggatgcccttccctcccaggggcactgacagcactggctgaaaggtctgaagagccagaggaggagccctgctggctggcccaggatggggcaaggagggagggaaagccaggggatggggagggacatgagatggagtttaaggcacacagcgagcgatggaggagggaggtgctggcctctcccctctgaattaactcccccaggagctcagctctggcctcagtttggtgaggttcagaagactcccagcaataaaaagtatttcttggatgatcaagtcctcccttactccagcctcctcttctcagctccccaggtggtgtgggaggggcccagtggcctggggtggggggtaaggggcgacgggatgacagagactgctgctgctctcaggcgggcaagggaggccctgatggcgccagtaccgcggggcagagcaccagctgcggggctgctaaggcgtcacctgcgtacctttccgggcctgctgaaaagctcacaccatcctccatgcatcagaaggggaagcggaaagtgaaaggatcctcccccgagtctactctgcattctgcccacccagctgcttgcccccattccagggcccctgcaggacaggccaccccaggaggcctccactcatttgagatttcagaagattcagggaccctggagcttagggagggggagcacccaccacttccttggtctgctgatgaggtctctgctgctctctccctggaggggagtgggtggaaggtcaagaggggagagatggaagtaaaagcagaaaacaaaaccaaaccagaaaaccaccggtttgtaaattggcaacaagacctgcctgctggctgccctgaggcccacgggtctgctcccacagaggaaggaggcaggaagcggctggcaggctccagctcccgcccggccccgctgagggctggccagcctcatggctccgaggccgggactcctgccatgcgcctaacaggtccaaggtcctctccggtctgggagctgccctctgcgcccctcgagcattctcctggatcccggcgtctgctcctaggtcttctcttcccggtctgtttttctccttgttatgttcctgggtttaattttcagagacagttcccatagggcctcctcagccaggtggtcactgaagtcattgaagaagtttataatgtcgtcgttcctccgcatgtcatagtgcgcctgctggaagcagcgcatgctgtcgaggatgttgaactgctgccaccgcttggagaagttcactttcccgtcgatgtagtctgggtttcccaggtgaacgaaggtcaggtcctgcaggatcagccccaggtacgggatgcacggcggttccacctccgagagggcggcccggtaggctcggaaggaggacgagctgtcgatcagtgtgcagtactcggccaggccctctgaagtctgcttctgccactccagcctgcggatgggcgccgagtccagggcagagaggatggccaagtaggagttgaagttattcagcttccgcaagtgcttcatgatcttgatgaacttcaagagcagccgttccctgtcctgggccttttcctgtaacatgattatggaccggacccagtaggacatgttgttgaagtgctccgtgaactgggtcaagttggggctcttctcctcattctgctcttttgcccaaagcaaaacctcaggaatctctattttatagaagagctcagcatccagcagcgttagctgctccgctatctcatggctgtgaaagtcgtgcaaggtccccggcctggctgctaccccccgggctgccaggggctggctggaggtggcacacctgagtagcttcttctggtccaccttgtccaggatgttcttccggagcacacgggccaggctcagctccccattgcacaccaggcggaagaccagttccatcagcagcttcaggatctcttctgtcaactccaccaggcagagctcatccaccacccgtaccagcacgaagaacgtgttcttgctgacgcgcttcttgaatgtgtcggcaaagggagagaatttctcatatctgtactgcagcttcttgatgagctcctctggggagatgaaggtcctgtaggtggtcaggaatgcctcgcagtacaacaccaaatctttcctgtcagtctcagtagcatggaccagtaagatgtccccagatcctccgcggacgtccggcccgtcatcaccctcctgcttgagcgtcagcctggacataatttcgttgtggtcaatgagggacagctcgtccacttcctcctccgactgagccgactccagagcatctggtgactttggggccctctcactgccgtctctgctgtccttcccagggacgccgctgaccgctgagggatctctgggatgtccgtctttcccagccggtggctctcctcgagagggagccagctcctcgctgctctggccagaggaatacagattgacatattcaccctcaccagcttcctcactggcgttttcactcgagtcagtgaaagaggtttcggaaggaaggcagacagtattcccatgaaagctgctctcctgagaagccgagagaggcccgtccacggtgctgggaggtggaccggccatggttggcacggctaagtcagagctctgagactggtgggcaggtgggaaatgtggagaggaagaggaggtaggcggaaggaaaggcggaacggaagcttggtggtgaggcacgaaatcctgggagtaggacctaaacacagacttatacgagggcacgggcaagctgccgtgccggctgagaaaggagttagagacggacacactgaggccctgagcggcactgccgtcctcgggggtgaaggccactttagtttgctggacacagtgggagacagaggagaaggaagaagcagcacaggaggcctgcagctgccgctgcttggggggtagggcgggcggcggggccagctcctgcacggagtccaccccactgaaggagtcgctgaagccgtatacctccatgaggagcttgttcttctgctggtagatgtgctcgttctgtggcgtctggtagaacatagagggctgcggctccgagtagtcctccagcaactgcatgtaggccagcatgtgtttgtttttcttctctggtagaggaggtggtttttctgggtcaccggttgactcaggagcagtaaaatcacccacaaattcgacaggggctgaggaacctccatgctgaaagggcagaatagcagcaaagggcgcgtaggggacggatgggatcggggctgtgctctgcaggtcctccccagagatgttgtcatactgcgagggatgccgctcgtaggacaccctgcagccagagccgtccgccgtctgggaggctgcgctcctgcgcttcttctcggggagagcaggtggcgtatctgtctgctgccctggggccagaggtccgtctggctggggatggccgccaagaggcagctggaaaggagggccaagaaatggagacccagactcccccaaagactctggcaacgggctaaggttccaggccgtctgctgaggtatctggtctgcgttagagaggtcttgctggaggaattcatagtcgggatcatagtggtctagtgtttcacagcttgtgttccgggagcactgcccactgtccctgtccagagaggacagctgctcgtctgacttgctgagcttgcctatgctgctgcagggggagaggcggggcgactctccaccatatgagtggctgcctcctgacagtcgcctctgtgcgtaacagtcaacatcaaaatcctgcctattgattccaacaggcaaactggagccactggtggctcggctcatgggggccaccacagccactcgggtaggggacggcgccgactgtcttttcttgggtggcaatgctggtggaggactattatcaaccacccgaatgccaggcagaggaggcttggggggcgcgacctcttcatccgtggcatctgggaggagctcagttgactgtgacatcccagtcgtcttgtttaggatctctacctcgcggtctgtcagggggagctctgctgggccatcaggcttgctggcaggggaactgggcttcacggggctcgtcggagacggacgtccctgcttctcgatggtgagcctgaccagctccttcactccatccagcacagccttgatgacccccttcacagtcgtcaccatctccttgtcttctgagttcacgccttccagcatcacttggtcagaccagcgaatgaggttggcgaggctttggtacactcggctatagcaggaagagagggctgagctgtgctgaattcgaggatcgttctgcaccaggggtaagatggcctccagcaccttgctggctgaccctggaagcatctccagtaccttcttatcaattgccattttgtccacaatggtcttaaagtagcgcagggcactgacaacttccttctctttctcctccagccagctcaggttcttctgcctttgagacctggaagccacagcactggtggacataaattctactgcctgctgctccagatccaaggggagagggtagccctctggtagaaatctgtctgttgcctctttgttcacaggcttctctggaatctttacggacacctcagctggttttcccttctttgatggcgttctcttgattttgggtgagtggaatttgtccatcagcttcatggtgaaggaagagagatgagaacgctgagagtctgctttctcgatcttgccggacatttccgggctgcgccggaggccgaggccgccgctcatcgggcccgggccgggccgccgcggggcgacaggggcggcgcgcccgccgctcgcctcggccctggctcgccacgcctcagacccgcgccggcatggcgggctccgcgcggccgcggccctgcgctcggcgaccgcgctccagcccgcccgggcccagccgctcccgccgcgcccgccgccgccgctccgcctcccgcgcgcccgccgccgctcccccggcccgcgagccggccgcagc

SEQ ID NO: 16470 - RNA, 5130 nt, Homo sapiens
  source 1..5130: mol_type = other RNA
gtcctaggaggctcctctgtggccaggcttctgcctccctgcaccctgagggaccattcgggtgcctcagggatgcccttccctcccaggggcactgacagcactggctgaaaggtctgaagagccagaggaggagccctgctggctggcccaggatggggcaaggagggagggaaagccaggggatggggagggacatgagatggagtttaaggcacacagcgagcgatggaggagggaggtgctggcctctcccctctgaattaactcccccaggagctcagctctggcctcagtttggtgaggttcagaagactcccagcaataaaaagtatttcttggatgatcaagtcctcccttactccagcctcctcttctcagctccccaggtggtgtgggaggggcccagtggcctggggtggggggtaaggggcgacgggatgacagagactgctgctgctctcaggcgggcaagggaggccctgatggcgccagtaccgcggggcagagcaccagctgcggggctgctaaggcgtcacctgcgtacctttccgggcctgctgaaaagctcacaccatcctccatgcatcagaaggggaagcggaaagtgaaaggatcctcccccgagtctactctgcattctgcccacccagctgcttgcccccattccagggcccctgcaggacaggccaccccaggaggcctccactcatttgagatttcagaagattcagggaccctggagcttagggagggggagcacccaccacttccttggtctgctgatgaggtctctgctgctctctccctggaggggagtgggtggaaggtcaagaggggagagatggaagtaaaagcagaaaacaaaaccaaaccagaaaaccaccggtttgtaaattggcaacaagacctgcctgctggctgccctgaggcccacgggtctgctcccacagaggaaggaggcaggaagcggctggcaggctccagctcccgcccggccccgctgagggctggccagcctcatggctccgaggccgggactcctgccatgcgcctaacaggtccaaggtcctctccggtctgggagctgccctctgcgcccctcgagcattctcctggatcccggcgtctgctcctaggtcttctcttcccggtctgtttttctccttgttatgttcctgggtttaattttcagagacagttcccatagggcctcctcagccaggtggtcactgaagtcattgaagaagtttataatgtcgtcgttcctccgcatgtcatagtgcgcctgctggaagcagcgcatgctgtcgaggatgttgaactgctgccaccgcttggagaagttcactttcccgtcgatgtagtctgggtttcccaggtgaacgaaggtcaggtcctgcaggatcagccccaggtacgggatgcacggcggttccacctccgagagggcggcccggtaggctcggaaggaggacgagctgtcgatcagtgtgcagtactcggccaggccctctgaagtctgcttctgccactccagcctgcggatgggcgccgagtccagggcagagaggatggccaagtaggagttgaagttattcagcttccgcaagtgcttcatgatcttgatgaacttcaagagcagccgttccctgtcctgggccttttcctgtaacatgattatggaccggacccagtaggacatgttgttgaagtgctccgtgaactgggtcaagttggggctcttctcctcattctgctcttttgcccaaagcaaaacctcaggaatctctattttatagaagagctcagcatccagcagcgttagctgctccgctatctcatggctgtgaaagtcgtgcaaggtccccggcctggctgctaccccccgggctgccaggggctggctggaggtggcacacctgagtagcttcttctggtccaccttgtccaggatgttcttccggagcacacgggccaggctcagctccccattgcacaccaggcggaagaccagttccatcagcagcttcaggatctcttctgtcaactccaccaggcagagctcatccaccacccgtaccagcacgaagaacgtgttcttgctgacgcgcttcttgaatgtgtcggcaaagggagagaatttctcatatctgtactgcagcttcttgatgagctcctctggggagatgaaggtcctgtaggtggtcaggaatgcctcgcagtacaacaccaaatctttcctgtcagtctcagtagcatggaccagtaagatgtccccagatcctccgcggacgtccggcccgtcatcaccctcctgcttgagcgtcagcctggacataatttcgttgtggtcaatgagggacagctcgtccacttcctcctccgactgagccgactccagagcatctggtgactttggggccctctcactgccgtctctgctgtccttcccagggacgccgctgaccgctgagggatctctgggatgtccgtctttcccagccggtggctctcctcgagagggagccagctcctcgctgctctggccagaggaatacagattgacatattcaccctcaccagcttcctcactggcgttttcactcgagtcagtgaaagaggtttcggaaggaaggcagacagtattcccatgaaagctgctctcctgagaagccgagagaggcccgtccacggtgctgggaggtggaccggccatggttggcacggctaagtcagagctctgagactggtgggcaggtgggaaatgtggagaggaagaggaggtaggcggaaggaaaggcggaacggaagcttggtggtgaggcacgaaatcctgggagtaggacctaaacacagacttatacgagggcacgggcaagctgccgtgccggctgagaaaggagttagagacggacacactgaggccctgagcggcactgccgtcctcgggggtgaaggccactttagtttgctggacacagtgggagacagaggagaaggaagaagcagcacaggaggcctgcagctgccgctgcttggggggtagggcgggcggcggggccagctcctgcacggagtccaccccactgaaggagtcgctgaagccgtatacctccatgaggagcttgttcttctgctggtagatgtgctcgttctgtggcgtctggtagaacatagagggctgcggctccgagtagtcctccagcaactgcatgtaggccagcatgtgtttgtttttcttctctggtagaggaggtggtttttctgggtcaccggttgactcaggagcagtaaaatcacccacaaattcgacaggggctgaggaacctccatgctgaaagggcagaatagcagcaaagggcgcgtaggggacggatgggatcggggctgtgctctgcaggtcctccccagagatgttgtcatactgcgagggatgccgctcgtaggacaccctgcagccagagccgtccgccgtctgggaggctgcgctcctgcgcttcttctcggggagagcaggtggcgtatctgtctgctgccctggggccagaggtccgtctggctggggatggccgccaagaggcagctggaaaggagggccaagaaatggagacccagactcccccaaagactctggcaacgggctaaggttccaggccgtctgctgaggtatctggtctgcgttagagaggtcttgctggaggaattcatagtcgggatcatagtggtctagtgtttcacagcttgtgttccgggagcactgcccactgtccctgtccagagaggacagctgctcgtctgacttgctgagcttgcctatgctgctgcagggggagaggcggggcgactctccaccatatgagtggctgcctcctgacagtcgcctctgtgcgtaacagtcaacatcaaaatcctgcctattgattccaacaggcaaactggagccactggtggctcggctcatgggggccaccacagccactcgggtaggggacggcgccgactgtcttttcttgggtggcaatgctggtggaggactattatcaaccacccgaatgccaggcagaggaggcttggggggcgcgacctcttcatccgtggcatctgggaggagctcagttgactgtgacatcccagtcgtcttgtttaggatctctacctcgcggtctgtcagggggagctctgctgggccatcaggcttgctggcaggggaactgggcttcacggggctcgtcggagacggacgtccctgcttctcgatggtgagcctgaccagctccttcactccatccagcacagccttgatgacccccttcacagtcgtcaccatctccttgtcttctgagttcacgccttccagcatcacttggtcagaccagcgaatgaggttggcgaggctttggtacactcggctatagcaggaagagagggctgagctgtgctgaattcgaggatcgttctgcaccaggggtaagatggcctccagcaccttgctggctgaccctggaagcatctccagtaccttcttatcaattgccattttgtccacaatggtcttaaagtagcgcagggcactgacaacttccttctctttctcctccagccagctcaggttcttctgcctttgagacctggaagccacagcactggtggacataaattctactgcctgctgctccagatccaaggggagagggtagccctctggtagaaatctgtctgttgcctctttgttcacaggcttctctggaatctttacggacacctcagctggttttcccttctttgatggcgttctcttgattttgggtgagtggaatttgtccatcagcttcatggtgaaggaagagagatgagaacgctgagagtctggaacgacacctcctgtcctcttgttctgttccaaggttgtcaggctgggacgaaatcccaagaaagaaatgggcatgtggtcactatcatagcagactgccagttagggacatcagaatatatttctctgtcctcaagttaggaagtgagaggacaaacctggccttctgtgttgtttcagccactaattggttttgtcaattaggcaaaacataatttctctaagcctcttttctcatccacaggcattagcctagt

SEQ ID NO: 16471 - RNA, 5140 nt, Homo sapiens
  source 1..5140: mol_type = other RNA
gtcctaggaggctcctctgtggccaggcttctgcctccctgcaccctgagggaccattcgggtgcctcagggatgcccttccctcccaggggcactgacagcactggctgaaaggtctgaagagccagaggaggagccctgctggctggcccaggatggggcaaggagggagggaaagccaggggatggggagggacatgagatggagtttaaggcacacagcgagcgatggaggagggaggtgctggcctctcccctctgaattaactcccccaggagctcagctctggcctcagtttggtgaggttcagaagactcccagcaataaaaagtatttcttggatgatcaagtcctcccttactccagcctcctcttctcagctccccaggtggtgtgggaggggcccagtggcctggggtggggggtaaggggcgacgggatgacagagactgctgctgctctcaggcgggcaagggaggccctgatggcgccagtaccgcggggcagagcaccagctgcggggctgctaaggcgtcacctgcgtacctttccgggcctgctgaaaagctcacaccatcctccatgcatcagaaggggaagcggaaagtgaaaggatcctcccccgagtctactctgcattctgcccacccagctgcttgcccccattccagggcccctgcaggacaggccaccccaggaggcctccactcatttgagatttcagaagattcagggaccctggagcttagggagggggagcacccaccacttccttggtctgctgatgaggtctctgctgctctctccctggaggggagtgggtggaaggtcaagaggggagagatggaagtaaaagcagaaaacaaaaccaaaccagaaaaccaccggtttgtaaattggcaacaagacctgcctgctggctgccctgaggcccacgggtctgctcccacagaggaaggaggcaggaagcggctggcaggctccagctcccgcccggccccgctgagggctggccagcctcatggctccgaggccgggactcctgccatgcgcctaacaggtccaaggtcctctccggtctgggagctgccctctgcgcccctcgagcattctcctggatcccggcgtctgctcctaggtcttctcttcccggtctgtttttctccttgttatgttcctgggtttaattttcagagacagttcccatagggcctcctcagccaggtggtcactgaagtcattgaagaagtttataatgtcgtcgttcctccgcatgtcatagtgcgcctgctggaagcagcgcatgctgtcgaggatgttgaactgctgccaccgcttggagaagttcactttcccgtcgatgtagtctgggtttcccaggtgaacgaaggtcaggtcctgcaggatcagccccaggtacgggatgcacggcggttccacctccgagagggcggcccggtaggctcggaaggaggacgagctgtcgatcagtgtgcagtactcggccaggccctctgaagtctgcttctgccactccagcctgcggatgggcgccgagtccagggcagagaggatggccaagtaggagttgaagttattcagcttccgcaagtgcttcatgatcttgatgaacttcaagagcagccgttccctgtcctgggccttttcctgtaacatgattatggaccggacccagtaggacatgttgttgaagtgctccgtgaactgggtcaagttggggctcttctcctcattctgctcttttgcccaaagcaaaacctcaggaatctctattttatagaagagctcagcatccagcagcgttagctgctccgctatctcatggctgtgaaagtcgtgcaaggtccccggcctggctgctaccccccgggctgccaggggctggctggaggtggcacacctgagtagcttcttctggtccaccttgtccaggatgttcttccggagcacacgggccaggctcagctccccattgcacaccaggcggaagaccagttccatcagcagcttcaggatctcttctgtcaactccaccaggcagagctcatccaccacccgtaccagcacgaagaacgtgttcttgctgacgcgcttcttgaatgtgtcggcaaagggagagaatttctcatatctgtactgcagcttcttgatgagctcctctggggagatgaaggtcctgtaggtggtcaggaatgcctcgcagtacaacaccaaatctttcctgtcagtctcagtagcatggaccagtaagatgtccccagatcctccgcggacgtccggcccgtcatcaccctcctgcttgagcgtcagcctggacataatttcgttgtggtcaatgagggacagctcgtccacttcctcctccgactgagccgactccagagcatctggtgactttggggccctctcactgccgtctctgctgtccttcccagggacgccgctgaccgctgagggatctctgggatgtccgtctttcccagccggtggctctcctcgagagggagccagctcctcgctgctctggccagaggaatacagattgacatattcaccctcaccagcttcctcactggcgttttcactcgagtcagtgaaagaggtttcggaaggaaggcagacagtattcccatgaaagctgctctcctgagaagccgagagaggcccgtccacggtgctgggaggtggaccggccatggttggcacggctaagtcagagctctgagactggtgggcaggtgggaaatgtggagaggaagaggaggtaggcggaaggaaaggcggaacggaagcttggtggtgaggcacgaaatcctgggagtaggacctaaacacagacttatacgagggcacgggcaagctgccgtgccggctgagaaaggagttagagacggacacactgaggccctgagcggcactgccgtcctcgggggtgaaggccactttagtttgctggacacagtgggagacagaggagaaggaagaagcagcacaggaggcctgcagctgccgctgcttggggggtagggcgggcggcggggccagctcctgcacggagtccaccccactgaaggagtcgctgaagccgtatacctccatgaggagcttgttcttctgctggtagatgtgctcgttctgtggcgtctggtagaacatagagggctgcggctccgagtagtcctccagcaactgcatgtaggccagcatgtgtttgtttttcttctctggtagaggaggtggtttttctgggtcaccggttgactcaggagcagtaaaatcacccacaaattcgacaggggctgaggaacctccatgctgaaagggcagaatagcagcaaagggcgcgtaggggacggatgggatcggggctgtgctctgcaggtcctccccagagatgttgtcatactgcgagggatgccgctcgtaggacaccctgcagccagagccgtccgccgtctgggaggctgcgctcctgcgcttcttctcggggagagcaggtggcgtatctgtctgctgccctggggccagaggtccgtctggctggggatggccgccaagaggcagctggaaaggagggccaagaaatggagacccagactcccccaaagactctggcaacgggctaaggttccaggccgtctgctgaggtatctggtctgcgttagagaggtcttgctggaggaattcatagtcgggatcatagtggtctagtgtttcacagcttgtgttccgggagcactgcccactgtccctgtccagagaggacagctgctcgtctgacttgctgagcttgcctatgctgctgcagggggagaggcggggcgactctccaccatatgagtggctgcctcctgacagtcgcctctgtgcgtaacagtcaacatcaaaatcctgcctattgattccaacaggcaaactggagccactggtggctcggctcatgggggccaccacagccactcgggtaggggacggcgccgactgtcttttcttgggtggcaatgctggtggaggactattatcaaccacccgaatgccaggcagaggaggcttggggggcgcgacctcttcatccgtggcatctgggaggagctcagttgactgtgacatcccagtcgtcttgtttaggatctctacctcgcggtctgtcagggggagctctgctgggccatcaggcttgctggcaggggaactgggcttcacggggctcgtcggagacggacgtccctgcttctcgatggtgagcctgaccagctccttcactccatccagcacagccttgatgacccccttcacagtcgtcaccatctccttgtcttctgagttcacgccttccagcatcacttggtcagaccagcgaatgaggttggcgaggctttggtacactcggctatagcaggaagagagggctgagctgtgctgaattcgaggatcgttctgcaccaggggtaagatggcctccagcaccttgctggctgaccctggaagcatctccagtaccttcttatcaattgccattttgtccacaatggtcttaaagtagcgcagggcactgacaacttccttctctttctcctccagccagctcaggttcttctgcctttgagacctggaagccacagcactggtggacataaattctactgcctgctgctccagatccaaggggagagggtagccctctggtagaaatctgtctgttgcctctttgttcacaggcttctctggaatctttacggacacctcagctggttttcccttctttgatggcgttctcttgattttgggtgagtggaatttgtccatcagcttcatggtgaaggaagagagatgagaacgctgagagtctgtgtccatggcagcacggtcgctcggtctggcagcctgggtagcttagaaactgtgctaggttagacaagcttctctgggagcaggcactttcatctacaaccccctagcagaaggcggtgcccagaaaaggcccaaggacaaactatgctgaaatgaactggcctcaggtctttctcccaaatagcagagaactcaaatgaagagtcatttcattcccagcggtttgggcagctcatgggatgacaggcaactttttcctttttttaa

SEQ ID NO: 16472 - RNA, 5062 nt, Homo sapiens
  source 1..5062: mol_type = other RNA
gtcctaggaggctcctctgtggccaggcttctgcctccctgcaccctgagggaccattcgggtgcctcagggatgcccttccctcccaggggcactgacagcactggctgaaaggtctgaagagccagaggaggagccctgctggctggcccaggatggggcaaggagggagggaaagccaggggatggggagggacatgagatggagtttaaggcacacagcgagcgatggaggagggaggtgctggcctctcccctctgaattaactcccccaggagctcagctctggcctcagtttggtgaggttcagaagactcccagcaataaaaagtatttcttggatgatcaagtcctcccttactccagcctcctcttctcagctccccaggtggtgtgggaggggcccagtggcctggggtggggggtaaggggcgacgggatgacagagactgctgctgctctcaggcgggcaagggaggccctgatggcgccagtaccgcggggcagagcaccagctgcggggctgctaaggcgtcacctgcgtacctttccgggcctgctgaaaagctcacaccatcctccatgcatcagaaggggaagcggaaagtgaaaggatcctcccccgagtctactctgcattctgcccacccagctgcttgcccccattccagggcccctgcaggacaggccaccccaggaggcctccactcatttgagatttcagaagattcagggaccctggagcttagggagggggagcacccaccacttccttggtctgctgatgaggtctctgctgctctctccctggaggggagtgggtggaaggtcaagaggggagagatggaagtaaaagcagaaaacaaaaccaaaccagaaaaccaccggtttgtaaattggcaacaagacctgcctgctggctgccctgaggcccacgggtctgctcccacagaggaaggaggcaggaagcggctggcaggctccagctcccgcccggccccgctgagggctggccagcctcatggctccgaggccgggactcctgccatgcgcctaacaggtccaaggtcctctccggtctgggagctgccctctgcgcccctcgagcattctcctggatcccggcgtctgctcctaggtcttctcttcccggtctgtttttctccttgttatgttcctgggtttaattttcagagacagttcccatagggcctcctcagccaggtggtcactgaagtcattgaagaagtttataatgtcgtcgttcctccgcatgtcatagtgcgcctgctggaagcagcgcatgctgtcgaggatgttgaactgctgccaccgcttggagaagttcactttcccgtcgatgtagtctgggtttcccaggtgaacgaaggtcaggtcctgcaggatcagccccaggtacgggatgcacggcggttccacctccgagagggcggcccggtaggctcggaaggaggacgagctgtcgatcagtgtgcagtactcggccaggccctctgaagtctgcttctgccactccagcctgcggatgggcgccgagtccagggcagagaggatggccaagtaggagttgaagttattcagcttccgcaagtgcttcatgatcttgatgaacttcaagagcagccgttccctgtcctgggccttttcctgtaacatgattatggaccggacccagtaggacatgttgttgaagtgctccgtgaactgggtcaagttggggctcttctcctcattctgctcttttgcccaaagcaaaacctcaggaatctctattttatagaagagctcagcatccagcagcgttagctgctccgctatctcatggctgtgaaagtcgtgcaaggtccccggcctggctgctaccccccgggctgccaggggctggctggaggtggcacacctgagtagcttcttctggtccaccttgtccaggatgttcttccggagcacacgggccaggctcagctccccattgcacaccaggcggaagaccagttccatcagcagcttcaggatctcttctgtcaactccaccaggcagagctcatccaccacccgtaccagcacgaagaacgtgttcttgctgacgcgcttcttgaatgtgtcggcaaagggagagaatttctcatatctgtactgcagcttcttgatgagctcctctggggagatgaaggtcctgtaggtggtcaggaatgcctcgcagtacaacaccaaatctttcctgtcagtctcagtagcatggaccagtaagatgtccccagatcctccgcggacgtccggcccgtcatcaccctcctgcttgagcgtcagcctggacataatttcgttgtggtcaatgagggacagctcgtccacttcctcctccgactgagccgactccagagcatctggtgactttggggccctctcactgccgtctctgctgtccttcccagggacgccgctgaccgctgagggatctctgggatgtccgtctttcccagccggtggctctcctcgagagggagccagctcctcgctgctctggccagaggaatacagattgacatattcaccctcaccagcttcctcactggcgttttcactcgagtcagtgaaagaggtttcggaaggaaggcagacagtattcccatgaaagctgctctcctgagaagccgagagaggcccgtccacggtgctgggaggtggaccggccatggttggcacggctaagtcagagctctgagactggtgggcaggtgggaaatgtggagaggaagaggaggtaggcggaaggaaaggcggaacggaagcttggtggtgaggcacgaaatcctgggagtaggacctaaacacagacttatacgagggcacgggcaagctgccgtgccggctgagaaaggagttagagacggacacactgaggccctgagcggcactgccgtcctcgggggtgaaggccactttagtttgctggacacagtgggagacagaggagaaggaagaagcagcacaggaggcctgcagctgccgctgcttggggggtagggcgggcggcggggccagctcctgcacggagtccaccccactgaaggagtcgctgaagccgtatacctccatgaggagcttgttcttctgctggtagatgtgctcgttctgtggcgtctggtagaacatagagggctgcggctccgagtagtcctccagcaactgcatgtaggccagcatgtgtttgtttttcttctctggtagaggaggtggtttttctgggtcaccggttgactcaggagcagtaaaatcacccacaaattcgacaggggctgaggaacctccatgctgaaagggcagaatagcagcaaagggcgcgtaggggacggatgggatcggggctgtgctctgcaggtcctccccagagatgttgtcatactgcgagggatgccgctcgtaggacaccctgcagccagagccgtccgccgtctgggaggctgcgctcctgcgcttcttctcggggagagcaggtggcgtatctgtctgctgccctggggccagaggtccgtctggctggggatggccgccaagaggcagctggaaaggagggccaagaaatggagacccagactcccccaaagactctggcaacgggctaaggttccaggccgtctgctgaggtatctggtctgcgttagagaggtcttgctggaggaattcatagtcgggatcatagtggtctagtgtttcacagcttgtgttccgggagcactgcccactgtccctgtccagagaggacagctgctcgtctgacttgctgagcttgcctatgctgctgcagggggagaggcggggcgactctccaccatatgagtggctgcctcctgacagtcgcctctgtgcgtaacagtcaacatcaaaatcctgcctattgattccaacaggcaaactggagccactggtggctcggctcatgggggccaccacagccactcgggtaggggacggcgccgactgtcttttcttgggtggcaatgctggtggaggactattatcaaccacccgaatgccaggcagaggaggcttggggggcgcgacctcttcatccgtggcatctgggaggagctcagttgactgtgacatcccagtcgtcttgtttaggatctctacctcgcggtctgtcagggggagctctgctgggccatcaggcttgctggcaggggaactgggcttcacggggctcgtcggagacggacgtccctgcttctcgatggtgagcctgaccagctccttcactccatccagcacagccttgatgacccccttcacagtcgtcaccatctccttgtcttctgagttcacgccttccagcatcacttggtcagaccagcgaatgaggttggcgaggctttggtacactcggctatagcaggaagagagggctgagctgtgctgaattcgaggatcgttctgcaccaggggtaagatggcctccagcaccttgctggctgaccctggaagcatctccagtaccttcttatcaattgccattttgtccacaatggtcttaaagtagcgcagggcactgacaacttccttctctttctcctccagccagctcaggtttttgttcacaggcttctctggaatctttacggacacctcagctggttttcccttctttgatggcgttctcttgattttgggtgagtggaatttgtccatcagcttcatggtgaaggaagagagatgagaacgctgagagtctgctttctcgatcttgccggacatttccgggctgcgccggaggccgaggccgccgctcatcgggcccgggccgggccgccgcggggcgacaggggcggcgcgcccgccgctcgcctcggccctggctcgccacgcctcagacccgcgccggcatggcgggctccgcgcggccgcggccctgcgctcggcgaccgcgctccagcccgcccgggcccagccgctcccgccgcgcccgccgccgccgctccgcctcccgcgcgcccgccgccgctcccccggcccgcgagccggccgcagcgcagcgac

SEQ ID NO: 16473 - RNA, 5026 nt, Homo sapiens
  source 1..5026: mol_type = other RNA
gtcctaggaggctcctctgtggccaggcttctgcctccctgcaccctgagggaccattcgggtgcctcagggatgcccttccctcccaggggcactgacagcactggctgaaaggtctgaagagccagaggaggagccctgctggctggcccaggatggggcaaggagggagggaaagccaggggatggggagggacatgagatggagtttaaggcacacagcgagcgatggaggagggaggtgctggcctctcccctctgaattaactcccccaggagctcagctctggcctcagtttggtgaggttcagaagactcccagcaataaaaagtatttcttggatgatcaagtcctcccttactccagcctcctcttctcagctccccaggtggtgtgggaggggcccagtggcctggggtggggggtaaggggcgacgggatgacagagactgctgctgctctcaggcgggcaagggaggccctgatggcgccagtaccgcggggcagagcaccagctgcggggctgctaaggcgtcacctgcgtacctttccgggcctgctgaaaagctcacaccatcctccatgcatcagaaggggaagcggaaagtgaaaggatcctcccccgagtctactctgcattctgcccacccagctgcttgcccccattccagggcccctgcaggacaggccaccccaggaggcctccactcatttgagatttcagaagattcagggaccctggagcttagggagggggagcacccaccacttccttggtctgctgatgaggtctctgctgctctctccctggaggggagtgggtggaaggtcaagaggggagagatggaagtaaaagcagaaaacaaaaccaaaccagaaaaccaccggtttgtaaattggcaacaagacctgcctgctggctgccctgaggcccacgggtctgctcccacagaggaaggaggcaggaagcggctggcaggctccagctcccgcccggccccgctgagggctggccagcctcatggctccgaggccgggactcctgccatgcgcctaacaggtccaaggtcctctccggtctgggagctgccctctgcgcccctcgagcattctcctggatcccggcgtctgctcctaggtcttctcttcccggtctgtttttctccttgttatgttcctgggtttaattttcagagacagttcccatagggcctcctcagccaggtggtcactgaagtcattgaagaagtttataatgtcgtcgttcctccgcatgtcatagtgcgcctgctggaagcagcgcatgctgtcgaggatgttgaactgctgccaccgcttggagaagttcactttcccgtcgatgtagtctgggtttcccaggtgaacgaaggtcaggtcctgcaggatcagccccaggtacgggatgcacggcggttccacctccgagagggcggcccggtaggctcggaaggaggacgagctgtcgatcagtgtgcagtactcggccaggccctctgaagtctgcttctgccactccagcctgcggatgggcgccgagtccagggcagagaggatggccaagtaggagttgaagttattcagcttccgcaagtgcttcatgatcttgatgaacttcaagagcagccgttccctgtcctgggccttttcctgtaacatgattatggaccggacccagtaggacatgttgttgaagtgctccgtgaactgggtcaagttggggctcttctcctcattctgctcttttgcccaaagcaaaacctcaggaatctctattttatagaagagctcagcatccagcagcgttagctgctccgctatctcatggctgtgaaagtcgtgcaaggtccccggcctggctgctaccccccgggctgccaggggctggctggaggtggcacacctgagtagcttcttctggtccaccttgtccaggatgttcttccggagcacacgggccaggctcagctccccattgcacaccaggcggaagaccagttccatcagcagcttcaggatctcttctgtcaactccaccaggcagagctcatccaccacccgtaccagcacgaagaacgtgttcttgctgacgcgcttcttgaatgtgtcggcaaagggagagaatttctcatatctgtactgcagcttcttgatgagctcctctggggagatgaaggtcctgtaggtggtcaggaatgcctcgcagtacaacaccaaatctttcctgtcagtctcagtagcatggaccagtaagatgtccccagatcctccgcggacgtccggcccgtcatcaccctcctgcttgagcgtcagcctggacataatttcgttgtggtcaatgagggacagctcgtccacttcctcctccgactgagccgactccagagcatctggtgactttggggccctctcactgccgtctctgctgtccttcccagggacgccgctgaccgctgagggatctctgggatgtccgtctttcccagccggtggctctcctcgagagggagccagctcctcgctgctctggccagaggaatacagattgacatattcaccctcaccagcttcctcactggcgttttcactcgagtcagtgaaagaggtttcggaaggaaggcagacagtattcccatgaaagctgctctcctgagaagccgagagaggcccgtccacggtgctgggaggtggaccggccatggttggcacggctaagtcagagctctgagactggtgggcaggtgggaaatgtggagaggaagaggaggtaggcggaaggaaaggcggaacggaagcttggtggtgaggcacgaaatcctgggagtaggacctaaacacagacttatacgagggcacgggcaagctgccgtgccggctgagaaaggagttagagacggacacactgaggccctgagcggcactgccgtcctcgggggtgaaggccactttagtttgctggacacagtgggagacagaggagaaggaagaagcagcacaggaggcctgcagctgccgctgcttggggggtagggcgggcggcggggccagctcctgcacggagtccaccccactgaaggagtcgctgaagccgtatacctccatgaggagcttgttcttctgctggtagatgtgctcgttctgtggcgtctggtagaacatagagggctgcggctccgagtagtcctccagcaactgcatgtaggccagcatgtgtttgtttttcttctctggtagaggaggtggtttttctgggtcaccggttgactcaggagcagtaaaatcacccacaaattcgacaggggctgaggaacctccatgctgaaagggcagaatagcagcaaagggcgcgtaggggacggatgggatcggggctgtgctctgcaggtcctccccagagatgttgtcatactgcgagggatgccgctcgtaggacaccctgcagccagagccgtccgccgtctgggaggctgcgctcctgcgcttcttctcggggagagcaggtggcgtatctgtctgctgccctggggccagaggtccgtctggctggggatggccgccaagaggcagctggaaaggagggccaagaaatggagacccagactcccccaaagactctggcaacgggctaaggttccaggccgtctgctgaggtatctggtctgcgttagagaggtcttgctggaggaattcatagtcgggatcatagtggtctagtgtttcacagcttgtgttccgggagcactgcccactgtccctgtccagagaggacagctgctcgtctgacttgctgagcttgcctatgctgctgcagggggagaggcggggcgactctccaccatatgagtggctgcctcctgacagtcgcctctgtgcgtaacagtcaacatcaaaatcctgcctattgattccaacaggcaaactggagccactggtggctcggctcatgggggccaccacagccactcgggtaggggacggcgccgactgtcttttcttgggtggcaatgctggtggaggactattatcaaccacccgaatgccaggcagaggaggcttggggggcgcgacctcttcatccgtggcatctgggaggagctcagttgactgtgacatcccagtcgtcttgtttaggatctctacctcgcggtctgtcagggggagctctgctgggccatcaggcttgctggcaggggaactgggcttcacggggctcgtcggagacggacgtccctgcttctcgatggtgagcctgaccagctccttcactccatccagcacagccttgatgacccccttcacagtcgtcaccatctccttgtcttctgagttcacgccttccagcatcacttggtcagaccagcgaatgaggttggcgaggctttggtacactcggctatagcaggaagagagggctgagctgtgctgaattcgaggatcgttctgcaccaggggtaagatggcctccagcaccttgctggctgaccctggaagcatctccagtaccttcttatcaattgccattttgtccacaatggtcttaaagtagcgcagggcactgacaacttccttctctttctcctccagccagctcaggtttttgttcacaggcttctctggaatctttacggacacctcagctggttttcccttctttgatggcgttctcttgattttgggtgagtggaatttgtccatcagcttcatggtgaaggaagagagatgagaacgctgagagtctggaacgacacctcctgtcctcttgttctgttccaaggttgtcaggctgggacgaaatcccaagaaagaaatgggcatgtggtcactatcatagcagactgccagttagggacatcagaatatatttctctgtcctcaagttaggaagtgagaggacaaacctggccttctgtgttgtttcagccactaattggttttgtcaattaggcaaaacataatttctctaagcctcttttctcatccacaggcattagcctagtcagcggttct

SEQ ID NO: 16474 - RNA, 217 nt, Homo sapiens
  source 1..217: mol_type = other RNA
gtcctccaggccatgagctgcggggccaggcgtggacaggcctgaaagggtcctcacgctcacagagggtccaggaaatgacaatacagccggagcgggactacaatgcgacaagtgaaggatgtgacagcctcgcattgcaactaccataccaataacaacccacttccgagtacagcgcccggcacacagcagcatgacgtcatttattcctctg

SEQ ID NO: 16475 - RNA, 35 nt, Homo sapiens
  source 1..35: mol_type = other RNA
gtgaaatgtttaggaccactagacccggcgggcgc

SEQ ID NO: 16476 - RNA, 1132 nt, Homo sapiens
  source 1..1132: mol_type = other RNA
gtgaaggcccggcggagacactctgcccaccccacaccctgcctatgggccacacagctgggcctgggtgctccaggagcatgagcccttctccaggccatggtgtctgcctgcagccactaggcgcctctcggtccccacacaaataaaggcactgatggatccaaagtcgggtgcacagcccagttgccatggagcctgctgtgttagcttggcacaagtcaccaaacctctgggctgtgctggtgcataaggtggtggactctgcagtccccacggccccttccggctctgccgttctctgtgcccatccagggccttccacttttgtggctggaggcaccaagctcccatacctttgtgtctgctgtggcgtacctgccacggatgggcatgctctgcgcatgcccacgatgttctgttcccgagcccgtgtagcaccgggcctgcagctggggcaggccgacgagcccagttagatggctggcagctccttgcagaaaacagaaggggtcagatggacaggaaggcgggctctgcgggcggccgaagggtggggcctggtggcggctgcccagccgacatcacatggtccggctgtactcgatgccactcttggaagagatgcccgaccatggcaggaagctgcagagcaggctgtgggcctggcggtagactctgtgcggaatggagcaggggctcaggctggctagtgcagagcccaggtgctggatgtagtccgtggggctctctttatgtattttggtcctgttcttaatttcagctactatcattcccacaatggcacctctgtaggttgcagcaagggaaaagaacttcttgttggatgtgatatcacgataccatgagtctgggtactcgatggggaaccagtcgccacacaggtgcttcacagtgtctatgtcatcgtggcagaggaggcgcaggctgacctcgctgagcgcgctggatggcaccacctctgtcattcacacctcgtgggggagccggcggccgctgggggtgttgtagggctcagcgcatcctggaggcgaagggagccgggaagtgggaccgcgcggagcccgcaacgagttatgtaaccggcaggggccgcagccgggacggaggc

SEQ ID NO: 16477 - RNA, 2087 nt, Homo sapiens
  source 1..2087: mol_type = other RNA
gtgactgataccttggaggcattttgtatatttggaaattctcatttgcatttttagacaatggagtaactcttttgcaggttgtactaaaacacaaacacaccactgaagaaaccagactaggaatttcagcattcattcgatgtttctgggacagggctccttcttgaatttaagttttgagaatccaaaatctcttctgtttgcccatctgcttctacctctattttgttctgaatctcttttgcatcttcactaaggcaagttcttatgctctcgtcctcctctaggactctctggactgtgatggcagcactcggagaactaacagtagtggcagcagcaggaacaatgactggagtgtgaggaggagaagctggaggagttggaggagttggaggaaaggaaggaactgtggaaggggtgatgggagctgggatacactccagtttcatttcttctgggggattttcgagaatctccaattcaagagtcaatggcaatacttcctgttttactatttccacaatgctctccgtggctgataatttttcgctaactccatttatttcattaattaggttagtactagaaaccagtggaatatcattaggtgctacactacagggtttcttgcatatatcatcatcattttcatttgttggtaaagggtctgatgtttctgtgcaagatgtgaggctgggtataggaattgtgtcttctcttggggatgagagttcacatctgtcatctatagcagtggtgaatattggttggctactaagagcagaagaggtgggggctgcaattgtacttcgagcaacagaagaaacagtggtaggtgatggaggcagaggaagctctgctatggatactattgcagtagtttcagatgtctggccttcttgttctttcttctctccactgaggactagcctaaggactggggaaggagactttaacactggatctggttttggcttctcctcttgcttctggtcgctagctgcagtgacaggggtgctggcagcaagatgagcgctctccacagtcccataaaccacagggctgtgctcggggacctggctgggcagctgctgaggaggagtaggtgtggacgtgggtcttcctatgggtggagtaggatttctgctgccacctccagacataatctcctctgttatgtctttacctccctggtttggatcccgaattcttatagtttttttctctctcttggctggaggcggctgttgctgcgtaggcactatgataggtgctgactgatacaccggctgacttgggtaaaaaggcgttccataagcattggggaagtccccaggtcctggtccaggataaaaaggacctggccccggtggttgaactggatattgttgggggggcccaacataaggagggccactatgacggtactgtggtatacagtactgaggcccctggggcactgggtacggcatgggcagatggttaaccatcatgatgtgctgattagcctggtacactgcagtgggtgtctgtgcaccaggacgaatggaaggactgctgttcgggatggtagctctaggaggctgtatttgaggcctctggaaaaactgatgatggggaggtcgaggccccgctgcaaacggagaacgggtttgaggttgtgaattcattgtctgaggggtttgagggtataccagcgtggttggacctgcattctgtccagagggataaggggtttgagagagtccaggggacgatgcatgtcccgggggcgttgccgcaagatttggatgccccttgtttatttcatgtgctgaataaggggatggggtaggggttcccggctgtcttgccacttgtgttaccgtgctgtagactgctgagacagcgggagtgaagattcgatcctcaagaggttgttgcacaggtcctctaggaattcttgggaaaatgatgtgatcgctccaaacttcagtttcctcatcaatactctgtgggattgtgataaaggtttgaacattcccctttgtaatgtgcagtcataacttctaagctaaaagccaaaggtgaaaaaatattcc

SEQ ID NO: 16478 - RNA, 963 nt, Homo sapiens
  source 1..963: mol_type = other RNA
gtgagacttctctcccttcagtctttgaaaagaagatagtgattctaagagcttcaaatggagtgatatggttggttgattttgtcaccatttttatggattgaaattatacagggtaatcttgaaaagatgcacaagtttcctgggagactcatctgtcaaaattcaaaagagaggatgggcaagagaggagaaactccagaggaggacacagaaagctgatgcatttagagtaaacactaagagcatctaagttctgccgtttggaggaagagagcggcttggggctaaacgcactttccagatgttatcttgcatagtgcctttcatgtagaaagtgtaagaattaggaatattgggcactaacggagggatacattaaagaaaagactgtctaagaagtatctctgtcttccctggtaacacttccacatacctgtagaaataatgttgtcctggctttaggacgttacgcttctgatcctgaatcctgtacatactggttgcttaggtggcctctgattaacaacgagccagctacactggccccattttcccctaaattatatgagatgggtggcccagtgatcttgcaggtaacttctggctccaagaaaaatgcacaacctaagtgaaggatctcagatcccaagcatactgcatgctgaaagtaactgcaatgttatcttaatatgatttctacatgtactatcttataacatggtacacaaaacattagaaaacttatgagaccacttgatcatctgagatgaggcctatcacttaaacactgcagtactgttatgcctatggtaatagtgttttctccataagagttttttttcctttccagatgcccatattttgaacaaattttgctccccaaaccatgatacttgtattttttttttgagatgggagttttgctcttgtctggagtgcaatggcgtgatcttggctcac

SEQ ID NO: 16479 - RNA, 209 nt, Homo sapiens
  source 1..209: mol_type = other RNA
gtgagacttctctcccttcagtctttgcagtttgtccatggcgctgtgctgcggcgctccgctgggactcgtagcgctcccccggtgcagggaggaccccgccgcagccgccgcgccctgccctcgtctgctctccggagtccgctcaggccgcccggctagccggctgtttgctgctcctgccgttgccatggcgacgggcaatgctc

SEQ ID NO: 16480 - RNA, 334 nt, Homo sapiens
  source 1..334: mol_type = other RNA
gtgagacttctctcccttcagtctttgcgttaaaactcgagtgacgctatgcttccagagctgtctcctcccaatcctaaacattgtagccgtgcatggacaggctggagtcagctcttccggaatggtcttctaactcctggcagacctgctcaacatccaacaggcttccaaatggaaagttttacttccattttactttcacgtttctaatttgcatgtattattcactacattcacagaataaaaattaaaactccacttataccactcaagtttttctcctagagtgtctgccctgggcctctcctctctctcgaagcctggtgttgtt

SEQ ID NO: 16481 - RNA, 66 nt, Homo sapiens
  source 1..66: mol_type = other RNA
gtgagccagtggaatggagagggcacagctcaggctctttcagcctcctccttggccagggcaggg

SEQ ID NO: 16482 - RNA, 58 nt, Homo sapiens
  source 1..58: mol_type = other RNA
gtgaggaggggctggcagggacccactccccaccattcggcgggactgggccccgcac

SEQ ID NO: 16483 - RNA, 1523 nt, Homo sapiens
  source 1..1523: mol_type = other RNA
gtgaggaggggctggcagggactgagctgcagacagcatcagaggggtgggggtcccacagggtcgggcaggggtagtcctgggtgtaaccggaagcagttgctgaccctctgcaggaggccggcaaacagcaggaagagctcggtcctggccaggcgctccccaacacagacgcggcggcctgcagagaaaggcaggaaggcctcccgcttcacaaagtgcccattcgcgtccaggaaatggccggggttgaactggcctggggtctgccactgtgtctcatccaggagcaccgaggtcagcaggggaatcacgggcgtgcccttggggagcaggaagccgcccagctgtgtgtcggccgcggtgcagcggggcacgtgcggcaggagcgtgatgaaccgctgcacctcgtggagcacggcgcttgtgtagggcagagcctgctggtcctccagccggggagtccgcccagggcccagcacgcggtctagctcctcctgcacccggccctgcacgtccgggtgccggcccatcagaagtgcggcccactgcagcgtggccgaggtcgtctccgtcccggccatgaccatgtccagggtgcaggccaccgcgttggcctcagcaaacaggccctcggggtcatccccctgtccctgctggatcagggcgtccacatagctgcacacggggtcccccgggcacacgtggggcctccgcgcctccaggagggtcctcagaatggcacggacctcctcgatcttgcgcaggacgggccggtgcagctggagcagggccccgagccatgggtagacgttgaacagctgcaggccaggggaccccaagaggaccatgacctcatcgatgagacccagcagggacacaaacacggggtcccggtagtcaaatcggcggccgaagaggagcgcgaaggtgatattggagggagcccagcccagtagggccagcgggaagggccggcctctgtagccatccagctgcccagagaggcatttcagctcctgcagaatcttgtcagccaccggctcccggcccacgcccaggctgtgcagggcacgcaccgtgaactggcgggcagccctccagcgcgccccagatgagaagaagatgcctccacctcgctggatgagctggaagatggcgatgggaggccggtcggccagctcctgcccggggcccgccagcgcctctttgaccgcctcgaaccccgtcagcaccaccgtcttctggcgccccaggtgcacggtgaacaccggcccgtagcgttctgagagctccatcagggaccggtcctgttgcgacagacgcagcaagtgcaggttcccgacgagcggcagcgggcgaggccccgggggccaccgggcagctggggaggggtcttgggcgcaggcgcagagcagcccccagagccccaggaggcccaggaacagcaagagcagcagggccatgaggacgtggctggtgaggctccactcccctcctgggccccgtcccccccgcaccct

SEQ ID NO: 16484 - RNA, 1750 nt, Homo sapiens
  source 1..1750: mol_type = other RNA
gtgaggaggggctggcagggactgagctgcagacagcatcagaggggtgggggtcccacagggtcgggcaggggtagtcctgggtgtaaccggaagcagttgctgaccctgtgggggtgggggtgagggtgggagtcctcagggccctcccagagcagtccgagctgtggggtgggaggagagagggtgggaggacccagggctgggaggggagtggtcaggaggacctgggggctgggggagctcctagggcctgggcaccgcacacagggcctgggccctcggcctcatggtaaaagcccgggcgggcgtggtgtccagggaggccggactgacgccaggcgggggcagcaggcggtacctctgcaggaggccggcaaacagcaggaagagctcggtcctggccaggcgctccccaacacagacgcggcggcctgcagagaaaggcaggaaggcctcccgcttcacaaagtgcccattcgcgtccaggaaatggccggggttgaactggcctggggtctgccactgtgtctcatccaggagcaccgaggtcagcaggggaatcacgggcgtgcccttggggagcaggaagccgcccagctgtgtgtcggccgcggtgcagcggggcacgtgcggcaggagcgtgatgaaccgctgcacctcgtggagcacggcgcttgtgtagggcagagcctgctggtcctccagccggggagtccgcccagggcccagcacgcggtctagctcctcctgcacccggccctgcacgtccgggtgccggcccatcagaagtgcggcccactgcagcgtggccgaggtcgtctccgtcccggccatgaccatgtccagggtgcaggccaccgcgttggcctcagcaaacaggccctcggggtcatccccctgtccctgctggatcagggcgtccacatagctgcacacggggtcccccgggcacacgtggggcctccgcgcctccaggagggtcctcagaatggcacggacctcctcgatcttgcgcaggacgggccggtgcagctggagcagggccccgagccatgggtagacgttgaacagctgcaggccaggggaccccaagaggaccatgacctcatcgatgagacccagcagggacacaaacacggggtcccggtagtcaaatcggcggccgaagaggagcgcgaaggtgatattggagggagcccagcccagtagggccagcgggaagggccggcctctgtagccatccagctgcccagagaggcatttcagctcctgcagaatcttgtcagccaccggctcccggcccacgcccaggctgtgcagggcacgcaccgtgaactggcgggcagccctccagcgcgccccagatgagaagaagatgcctccacctcgctggatgagctggaagatggcgatgggaggccggtcggccagctcctgcccggggcccgccagcgcctctttgaccgcctcgaaccccgtcagcaccaccgtcttctggcgccccaggtgcacggtgaacaccggcccgtagcgttctgagagctccatcagggaccggtcctgttgcgacagacgcagcaagtgcaggttcccgacgagcggcagcgggcgaggccccgggggccaccgggcagctggggaggggtcttgggcgcaggcgcagagcagcccccagagccccaggaggcccaggaacagcaagagcagcagggccatgaggacgtggctggtgaggctccactcccct

SEQ ID NO: 16485 - RNA, 140 nt, Homo sapiens
  source 1..140: mol_type = other RNA
gtgagggcatgcaggcctggatggggaccccaacggggagtccggggcagcacgtcacaatgccatgtccattccgcccaccccccaagctgcaggaccacagctgataacctctcaactttggcccagccaccccgact

SEQ ID NO: 16486 - RNA, 875 nt, Homo sapiens
  source 1..875: mol_type = other RNA
gtgagggcatgcaggcctggatggggactctctttccctttatctcaacaggcgaatgaaagaagttgagggtttttcctgtgtgttattaatcacgcgaacctgaatttggccccagctccactagacactgtgacctttggcatgttatttcatttctctgagcctcagtcttggcacctcgtgatctgcccgccttggcctcccaaagtgctgggattacaggcgtgagccacagtgcccggccaattcactgcttctttaagattctcctgtagcccattttccagaaaacaatgatgctgtatgtatatatgtcacctctggcaattgcaagagcatttaatgaatttcacatcaccatttccagtcagtcttgatgttccatttttgtttgtcaatctgtgcagatgttcaaaacaggatattctgattcttgtccaattcagtgtgaaaatttacagaagcatattgttatattgttagaagggaagttatgaagccatcccagccagttctgctgcaagccaggtgcacacccaaaaccataaggtcatgatggtcagatgagaaaatggaagtgaaaggacctgatgaactgtcactgaggcaaattaagttattaccatccagtgtcattcagctccacttggttaccctcgtctccaaataatttgccttaaaacagacatcattaacatctgtcttcagtggttattgagctcatttctgcagaaagcacctgaaggatgcagcccctgtctgtaatagtggctttctatccctagctgggggaagcagagatagagtttgaaatgacccactggtaagaaccagagatcttaatgtaaagaaaataaatgagcaaattttgg

SEQ ID NO: 16487 - RNA, 1045 nt, Homo sapiens
  source 1..1045: mol_type = other RNA
gtgagggcatgcaggcctggatggggactctctttccctttatctcaacaggcgaatgaaagaagttgagggtttttcctgtgtgttattaatcacgcgaacctgaatttggccccagctccactagacactgtgacctttggcatgttatttcatttctctgagcctcagtcttggcacctcgtgatctgcccgccttggcctcccaaagtgctgggattacaggcgtgagccacagtgcccggccaattcactgcttctttaagattctcctgtagcccattttccagaaaacaatgatgctgtatgtatatatgtcacctctggcaattgcaagagcatttaatgaatttcacatcaccatttccagtcagtcttgatgttccatttttgtttgtcaatctgtgcagatgttcaaaacaggatattctgattcttgtccaattcagtgtgaaaatttacagaagcatattgttatattgttagaagggaagttatgaagccatcccagccagttctgctgcaagccaggtgcacacccaaacttgagccccatgtccttggcaaaatggcgaaaacaaggcacttgcacttaaatgacccaagttaaaagttcctcttaggtgtttgaccttagatatatggtatagctgctccaaacccagatttcccctctgaagaaaagaaaaaagggaagtaatcatttttacttacaccataaggtcatgatggtcagatgagaaaatggaagtgaaaggacctgatgaactgtcactgaggcaaattaagttattaccatccagtgtcattcagctccacttggttaccctcgtctccaaataatttgccttaaaacagacatcattaacatctgtcttcagtggttattgagctcatttctgcagaaagcacctgaaggatgcagcccctgtctgtaatagtggctttctatccctagctgggggaagcagagatagagtttgaaatgacccactggtaagaaccagagatcttaatgtaaagaaaataaatgagcaaattttgg

SEQ ID NO: 16488 - RNA, 904 nt, Homo sapiens
  source 1..904: mol_type = other RNA
gtgagggcatgcaggcctggatggggactctctttccctttatctcaacaggcgaatgaaagaagttgagggtttttcctgtgtgttattaatcacgcgaacctgaatttggccccagctccactagacactgtgacctttggcatgttatttcatttctctgagcctcagtcttggcacctctggcaattgcaagagcatttaatgaatttcacatcaccatttccagtcagtcttgatgttccatttttgtttgtcaatctgtgcagatgttcaaaacaggatattctgattcttgtccaattcagtgtgaaaatttacagaagcatattgttatattgttagaagggaagttatgaagccatcccagccagttctgctgcaagccaggtgcacacccaaacttgagccccatgtccttggcaaaatggcgaaaacaaggcacttgcacttaaatgacccaagttaaaagttcctcttaggtgtttgaccttagatatatggtatagctgctccaaacccagatttcccctctgaagaaaagaaaaaagggaagtaatcatttttacttacaccataaggtcatgatggtcagatgagaaaatggaagtgaaaggacctgatgaactgtcactgaggcaaattaagttattaccatccagtgtcattcagctccacttggttaccctcgtctccaaataatttgccttaaaacagacatcattaacatctgtcttcagtggttattgagctcatttctgcagaaagcacctgaaggatgcagcccctgtctgtaatagtggctttctatccctagctgggggaagcagagatagagtttgaaatgacccactggtaagaaccagagatcttaatgtaaagaaaataaatgagcaaattttgg

SEQ ID NO: 16489 - RNA, 984 nt, Homo sapiens
  source 1..984: mol_type = other RNA
gtgagggcatgcaggcctggatggggactctctttccctttatctcaacaggcgaatgaaagaagttgagggtttttcctgtgtgttattaatcacgcgaacctgaatttggccccagctccactagacactgtgacctttggcatgttatttcatttctctgagcctcagtcttggcaccttgagccccatgtccttggcaaaatggcgaaaacaaggcacttgcacttaaatgacccaagttaaaagttcctcttaggtgtttgaccttagatatatggtatagctgctccaaacccagatttcccctctgttctggagtcagcactgtgttagatgacaagtcaggagtgagccagaaggaaacagtcactgtctcatggcatctgcattccaggccctcggagccactgcacacggaaaagccatcgaaggaaggggatctcctccccactagacacatgcactgctacaatttcaaagagcgctgggttctggacttcatggcatctcagttctttccttcttactactcatcatgtgattgttctcattttctatttcctaatctgtgaaattaaaggccaaaatgagttatctaaggatcctttcaattccagaataacacaattttttgactttaggaaaatgtgtctcggtttccatatttctaaaagagaaatgatgatattttccttgctagtacaactagctgtttctgaaattgaattcagataatatgtgaatgagttttaacaatataaagagtccatgtaaacttaagattctacgaagactatgattaggatatcatcattaatatgggacaaaaaagggcagccttgccatttccgcttgaggacgcagaatacactctggtcacttaaactgaaagcatggagatacctgcccccatgcaggtggctgacgtagcctgcaaatattaagaactcttacttctagagaagctcccccaccaaaatg

SEQ ID NO: 16490 - RNA, 831 nt, Homo sapiens
  source 1..831: mol_type = other RNA
gtgagggcatgcaggcctggatggggactctctttccctttatctcaacaggcgaatgaaagaagttgagggtttttcctgtgtgttattaatcacgcgaacctgaatttggccccagctccactagacactgtgacctttggcatgttatttcatttctctgagcctcagtcttggcacttgtcaatctgtgcagatgttcaaaacaggatattctgattcttgtccaattcagtgtgaaaatttacagaagcatattgttatattgttagaagggaagttatgaagccatcccagccagttctgctgcaagccaggtgcacacccaaacttgagccccatgtccttggcaaaatggcgaaaacaaggcacttgcacttaaatgacccaagttaaaagttcctcttaggtgtttgaccttagatatatggtatagctgctccaaacccagatttcccctctgaagaaaagaaaaaagggaagtaatcatttttacttacaccataaggtcatgatggtcagatgagaaaatggaagtgaaaggacctgatgaactgtcactgaggcaaattaagttattaccatccagtgtcattcagctccacttggttaccctcgtctccaaataatttgccttaaaacagacatcattaacatctgtcttcagtggttattgagctcatttctgcagaaagcacctgaaggatgcagcccctgtctgtaatagtggctttctatccctagctgggggaagcagagatagagtttgaaatgacccactggtaagaaccagagatcttaatgtaaagaaaataaatgagcaaattttgg

SEQ ID NO: 16491 - RNA, 855 nt, Homo sapiens
  source 1..855: mol_type = other RNA
gtgagggcatgcaggcctggatggggactctctttccctttatctcaacaggcgaatgaaagaagttgagggtttttcctgtgtgttattaatctgaatttggccccagctccactagacactgtgacctttggcatgttatttcatttctctgagcctcagtcttggcaccatttccagtcagtcttgatgttccatttttgtttgtcaatctgtgcagatgttcaaaacaggatattctgattcttgtccaattcagtgtgaaaatttacagaagcatattgttatattgttagaagggaagttatgaagccatcccagccagttctgctgcaagccaggtgcacacccaaacttgagccccatgtccttggcaaaatggcgaaaacaaggcacttgcacttaaatgacccaagttaaaagttcctcttaggtgtttgaccttagatatatggtatagctgctccaaacccagatttcccctctgaagaaaagaaaaaagggaagtaatcatttttacttacaccataaggtcatgatggtcagatgagaaaatggaagtgaaaggacctgatgaactgtcactgaggcaaattaagttattaccatccagtgtcattcagctccacttggttaccctcgtctccaaataatttgccttaaaacagacatcattaacatctgtcttcagtggttattgagctcatttctgcagaaagcacctgaaggatgcagcccctgtctgtaatagtggctttctatccctagctgggggaagcagagatagagtttgaaatgacccactggtaagaaccagagatcttaatgtaaagaaaataaatgagcaaattttgg

SEQ ID NO: 16492 - RNA, 1036 nt, Homo sapiens
  source 1..1036: mol_type = other RNA
gtgagggcatgcaggcctggatggggactctctttccctttatctcaacaggcgaatgaaagaagttgagggtttttcctgtgtgttattaatctgaatttggccccagctccactagacactgtgacctttggcatgttatttcatttctctgagcctcagtcttggcacctcgtgatctgcccgccttggcctcccaaagtgctgggattacaggcgtgagccacagtgcccggccaattcactgcttctttaagattctcctgtagcccattttccagaaaacaatgatgctgtatgtatatatgtcacctctggcaattgcaagagcatttaatgaatttcacatcaccatttccagtcagtcttgatgttccatttttgtttgtcaatctgtgcagatgttcaaaacaggatattctgattcttgtccaattcagtgtgaaaatttacagaagcatattgttatattgttagaagggaagttatgaagccatcccagccagttctgctgcaagccaggtgcacacccaaacttgagccccatgtccttggcaaaatggcgaaaacaaggcacttgcacttaaatgacccaagttaaaagttcctcttaggtgtttgaccttagatatatggtatagctgctccaaacccagatttcccctctgaagaaaagaaaaaagggaagtaatcatttttacttacaccataaggtcatgatggtcagatgagaaaatggaagtgaaaggacctgatgaactgtcactgaggcaaattaagttattaccatccagtgtcattcagctccacttggttaccctcgtctccaaataatttgccttaaaacagacatcattaacatctgtcttcagtggttattgagctcatttctgcagaaagcacctgaaggatgcagcccctgtctgtaatagtggctttctatccctagctgggggaagcagagatagagtttgaaatgacccactggtaagaaccagagatcttaatgtaaagaaaataaatgagcaaattttgg

SEQ ID NO: 16493 - RNA, 725 nt, Homo sapiens
  source 1..725: mol_type = other RNA
gtgagggcatgcaggcctggatggggactctctttccctttatctcaacaggcgaatgaaagaagttgagggtttttcctgtgtgttattaatctgaatttggccccagctccactagacactgtgacctttggcatgttatttcatttctctgagcctcagtcttggcacctctggcaattgcaagagcatttaatgaatttcacatcaccatttccagtcagtcttgatgttccatttttgtttgtcaatctgtgcagatgttcaaaacaggatattctgattcttgtccaattcagtgtgaaaatttacagaagcatattgttatattgttagaagggaagttatgaagccatcccagccagttctgctgcaagccaggtgcacacccaaaaccataaggtcatgatggtcagatgagaaaatggaagtgaaaggacctgatgaactgtcactgaggcaaattaagttattaccatccagtgtcattcagctccacttggttaccctcgtctccaaataatttgccttaaaacagacatcattaacatctgtcttcagtggttattgagctcatttctgcagaaagcacctgaaggatgcagcccctgtctgtaatagtggctttctatccctagctgggggaagcagagatagagtttgaaatgacccactggtaagaaccagagatcttaatgtaaagaaaataaatgagcaaattttgg

SEQ ID NO: 16494 - RNA, 895 nt, Homo sapiens
  source 1..895: mol_type = other RNA
gtgagggcatgcaggcctggatggggactctctttccctttatctcaacaggcgaatgaaagaagttgagggtttttcctgtgtgttattaatctgaatttggccccagctccactagacactgtgacctttggcatgttatttcatttctctgagcctcagtcttggcacctctggcaattgcaagagcatttaatgaatttcacatcaccatttccagtcagtcttgatgttccatttttgtttgtcaatctgtgcagatgttcaaaacaggatattctgattcttgtccaattcagtgtgaaaatttacagaagcatattgttatattgttagaagggaagttatgaagccatcccagccagttctgctgcaagccaggtgcacacccaaacttgagccccatgtccttggcaaaatggcgaaaacaaggcacttgcacttaaatgacccaagttaaaagttcctcttaggtgtttgaccttagatatatggtatagctgctccaaacccagatttcccctctgaagaaaagaaaaaagggaagtaatcatttttacttacaccataaggtcatgatggtcagatgagaaaatggaagtgaaaggacctgatgaactgtcactgaggcaaattaagttattaccatccagtgtcattcagctccacttggttaccctcgtctccaaataatttgccttaaaacagacatcattaacatctgtcttcagtggttattgagctcatttctgcagaaagcacctgaaggatgcagcccctgtctgtaatagtggctttctatccctagctgggggaagcagagatagagtttgaaatgacccactggtaagaaccagagatcttaatgtaaagaaaataaatgagcaaattttgg

SEQ ID NO: 16495 - RNA, 822 nt, Homo sapiens
  source 1..822: mol_type = other RNA
gtgagggcatgcaggcctggatggggactctctttccctttatctcaacaggcgaatgaaagaagttgagggtttttcctgtgtgttattaatctgaatttggccccagctccactagacactgtgacctttggcatgttatttcatttctctgagcctcagtcttggcacttgtcaatctgtgcagatgttcaaaacaggatattctgattcttgtccaattcagtgtgaaaatttacagaagcatattgttatattgttagaagggaagttatgaagccatcccagccagttctgctgcaagccaggtgcacacccaaacttgagccccatgtccttggcaaaatggcgaaaacaaggcacttgcacttaaatgacccaagttaaaagttcctcttaggtgtttgaccttagatatatggtatagctgctccaaacccagatttcccctctgaagaaaagaaaaaagggaagtaatcatttttacttacaccataaggtcatgatggtcagatgagaaaatggaagtgaaaggacctgatgaactgtcactgaggcaaattaagttattaccatccagtgtcattcagctccacttggttaccctcgtctccaaataatttgccttaaaacagacatcattaacatctgtcttcagtggttattgagctcatttctgcagaaagcacctgaaggatgcagcccctgtctgtaatagtggctttctatccctagctgggggaagcagagatagagtttgaaatgacccactggtaagaaccagagatcttaatgtaaagaaaataaatgagcaaattttgg

SEQ ID NO: 16496 - RNA, 253 nt, Homo sapiens
  source 1..253: mol_type = other RNA
gtgagggcatgcaggcctggatggggtgacaggagcagtggcctcagggcttagccctgggggcaactctggtttactcttgaaaaacttcacatacttgttttcatatactgggacctcctcctggggcacatatccttctttcaccctccgctgcttgcgccaggtcccgtcaggtcgctgtgttgacgcgatatacttgccgccggtctcgtcagtaacatagggagtcgccatcttgaaaacgcaaacc

SEQ ID NO: 16497 - RNA, 373 nt, Homo sapiens
  source 1..373: mol_type = other RNA
gtgagggcatgcaggcctggatggggtgacaggagcagtggcctcagggcttagccctgggggcaactctggtttactcttgaaaaacttcacatacttgttttcatatactgggacctcctcctggggcacatatccttctttcaccctccgctgcttgcgccaggtcccgtcaggtcgctgtgttgacgcgatatacttgcctgtctccgtagccgcagggctgccggcagcttccatggccgaagaggcagcggaccaggttgggcgggcggccctggcctggctctgccccgctgggcggcgccggggattcggcggcgaagtgatgagggccctagttgcttctcgcccagacctcctaaccctgagt

SEQ ID NO: 16498 - RNA, 6006 nt, Homo sapiens
  source 1..6006: mol_type = other RNA
gtgagtcagggtggggctgggtgggagggatgagcacagctgcaccctacccaactcaccccaacccccagtcaccctctggcccacactgctccccacacctctgcccaggtctcataaatcctgcccagtggcccctccccacacagccccccaagagcagttccacttgggattgtcatggtacctgcagctcagcaagctgacatctgtgcttcccaccccaacaggggcagggagcccggatgaagaaagaatgagggcagagggcaccccatgcccaagacccacccaccccaggaccctccaagaggccatcagggcgacgccaacacacacacagacacacacacacacacacaaacaaacacacaattacaccccacagtgtggtcacttacaggaggtgagccttttccactggtgggtcaggcctcagtggggtcactgagaacccaccaaatcctcccaaatcccagcgtcagggctctgttggtctcgctccagttcaatccctctctccctctctctctgcagcttatcctgtctccgtatctttccccctcattctcggagtcactcagtctccctcttaaacaacaggtctctctcccactccacctcccaccatctctcccaatctctctcattcattttctgaaatattcaatccctttcacacacgactttctccgtctctctcattgatacacacactctccccccatccctgtctctctctcacacacacacacatgcacacacacacgcacacaggcagactcagccctccagggtctatgtctctgagctgagccccgctgagaggcaggcttgtctggggattgcagggagcactcacgcccacataggatgtgtccacgtggacagcgcttggccctttatgtacccactgtggatccttcactaggcaaccaggctggacttggaccagtgcaggtggaactaagccaagaccctgaaggccagggcagggtcagctccagcctcagcactcgccctaatccaggcacggtggagagtagcgtgagccaccaggcgggcccaagctgaagagctcaccgcatagcggggacagggatggcaggagacttgccactcagaccagggaaggatgacagggaccccaggcacaggcacaggtgtcagcagagaccacatcagtgggggtccccttgggcaggtggggggtggcatccagggctggagggtcacaggccactggcatggctcagcccagttctcacacagcatcctccatctctataatcatggggtcagtgtcacccctgggcatgaaatggagatactgctgttggcaaatgagcttggagagcagaggccaagacttctgggtgtcaagtgaggtgtcacaactggggcctgacttcatagaggccaaggtttcttcatagaggaagaaaccccgggagagtggctcccacggagggaactgccatgcacagctccgggggaggaggtggagcagtggccaccagccctgacagaaggcaatgcggggcccaggggcccagaaagaaagggcagagtgtggcctggtgaggccactgccccaagggcctatgcagtcccttgactgcgacctttgacaaagtgtgttacttgggtggggttggggggactccaagctgtgatgactcaggccagctggcaggagcgtgcatggtgaccgggatggagcagggttcagtgaagcaaccccatggatataagcacagggcccaccatggcacatgcaaaggaaggggaggagaaggaccgggttggcaacaaggagaaacccggctcaaagcaggtttgagggaggaagcagagaggacagttcagaggacagctttgcaactgaccagttagaaggcaaaggagcccaggccaggcacggtggctcaagcctgtaatcccaacactctgggaggccaaggtgggctcgcttgaggtcaggagtttgacaccaacctggccaacatgctgaaaccccctctcaactaaaaatacaaaaagtaaggccaggcacagtggctcacgcctgtaatcccagaactttggaaggtcaaggcggatggatcgcttgaggccaggagttccagaccagtctggccaacatggtgaaaccccgactctactaaaaatacaaaaattagccaggcctggtggcgcacacttgtaatcccagcacttggaaggctgaggcagaatgcttgaacgtgggaggcagaggttgcagtcagcccagatcacgccactgcactccagcctgggcgacagagctagactctgtctttaaaaaaaaaaaaaaaaaaaatagctgggcgtcatggggcacacctgtagtctcagctactggggaggctgaggcatgagaattacttgaaccctggaggcagaggttgcagtaggcccagattgtgccaacgcactccagcctgggcgacagaacgagaccctgtctcaaaaaaaaaaaaaaaaaaagccgggcacagtggtacacacctgtaatcccagcactttgggaggctgaggtgggtggatcgcccctgaggtcagcagttggagaccagcctgaccaacatggtgaaaccccatctctactaaaaatacaaaattagccgggcgtggtggcgtgcgcctgtagtcccagctactcgggagactaaagcaggagaattgcttgaacccgggaggcggaggctgcagtgagccaagattgtgccactgcactccagcctgggtgacacaatgacactccgtctcaaaaaaaaaaaaagaaaagaaaagaaaaagcagctcagctagcaggagagagccagcaccggagcctccacgcctggactttactctctggccccagtgggatcacctcctccaagaagtggcccctggtcctgctgaaggccccactctaagatgcagcgctctccacgctgtgtaagtccctggctaaggctccctgaccacccctgtacttgccggctcagcccaccaggtggcgcccgcgccatgcctcggccctgctggactccgaagccgccacttccctgcgggcgcctcctggtgtttgttcccttgggctcggcctggacagccctgctggttcccggagcctagcccagccccgcgagtgattcacagaactcacacctgacggtgggggaggaaggggagagcagcagccaagaggtgggtccaggctctcccaggggcgagtgacttcagtccagatgtcccctgaacccctggggattccgcatcaggaccagggcctcccatgtccagaccccacattcccgtcagtgtgtcccggggagcacggagggacctccacactgcatttcatggggcgaccgcccttaacacccggacacacacggaaccccacactaccctaaagtctgaaaggtggacacgcgtggcgaagttttagaggaatttcaggacaaaagtcctgaaaccacaaggttcttaccacctgaaaaccagctccgtaacagacaaactagacacttgtgagtttgccggcatttgctttaaaaataacaaggctggtccaagatcttagaagaaaattatattcttttaaagaaaatgaaaatatcctcaagggaaaaacttaatttaagtcaaatcttgtccttttgtcgtggagccccttgccccgcgcgcagacacaggctttcctgaagcgtggccagggcgcccctctcatcgctcctgagcgtgacccggggctggagccgcacggggattttcccgagctgagcaggggggtcggggggcccaagccaggagccctggaagagggagcagggcggcaactggggccgcaaacacccatcaaagtccccaggaccaattcccacagacaccacgtggccacaggcagtgccctttgcaggccccctccccaagggtgtcacccctcaccccctcctgggaccccgcctaaaccaggcacccttccacccaccagcaggaactgcgctaggagatgcaggaacacccatgtccccgccagccccgccttccagaccacaccctgcccgggagtgcgctttgcgaggtcggggtcgggggggagggcgggggccaggcccctgaacaacagacagcagctcccacccagcaatgcagccgggtcacctcgcacccctggccaaggcaggggccctctccagcctggtgacccacggcctaccctgaggctgcagggcacagggggcctccaagtggaaagctggtgatggggtgggtgggaggcagggcccgcagggaagtgacttgagcaggcacagacggtgaataaatagaagcttccacgcgggggtccggcccctgcagacagcagctcggtgggaaactgattggagggagctcccctgacgctgaccagggccacccacgcgggccctccctccacacccacacccaccccggcccagggacgggttttcccctgctcagagctcagtgacgtgcacagtgggtgagggaagaggcccaggttggaggcgccgcaggtggcaacgacgacacagtaggtggcccgccaggggatagcaacggcgtccctcctccccgctcagctgcagcccgcagtcctcacagtggtaacatgccacgtggtagtctctgtccatggacaccacacggatggttgtctcgcagccctgtgcagggaggataggacgggcacaggaggcgcattttggtgcaaaaaccgtgtgatagtctcgcacgcagtagatgttgttctccacgtccacggtgaagggaaccccgtccaggcactcattgcacacggagcaccggaagcagcctgggtggtaggacttgcccagggcctgcaggatcatttccatgatgagatgtccacacacgctgcatttgtcggccgtctgctggaacccggagtacaggaagtcctcctggcagtacactttctcacccacgttgtagaacgccttcccacggagtcgtctcccacacgagtcgcaggtgaagcagtcagtgtgataaagactccccattgcctggcacgcctgctgggctccgtagatgccaagcccacacttgatgcaaatgccgaagtagtcccgcgccgtgcgcgcctcgagcgcccgctccagctcccgggtgagcgcctccagccgccgctcggccgcgcttgggccgccctcccggccagggggcagcgggagtgcaggcagcgggaagggagccggccccgcaggctccggggagcgagcgggcgcggggcaggcgccgggcgggaggaagtcagcgtaggcgccggccgagccccgggagccgaggctggaaacgctggagcgggcgctgcccaccgaaggcggcccgggaccgggacgcgggtccgagcgaccggagcgcgggctgccgtggcgctggtcgtagcccaggctgatgccgctggatcgggcgctgccgccaccgccgccgccgtcggaccccgccaggctggcccgtgggctgcccgcaggctgcgcgctgagctccggaaccgccgcgcgccggggaccccgctccccgcggctcagtccgtccgccccggcctcggggccgccgctgcccttccctctgcggcccagcgcgggcgccgcctcgtctccaggcccaggccgcggcccccgccgcccccgaccgggagagccgcacccgggctccagctcccgcagggccagcccggccaggagtagggccgcctcgtccgcgcccgccctggagcgctgcatggcccggcccgccggccctggcgcgtcacctccgcctccgcttcccgccgccgctccggccgggccgccgcatcgtccgcccgaagcccggagcccgccccgggacccctgggcgcggggcggggcggggccggcgccgggccggggtcgttccggcggccacgcgcgggccgggggacgcggcgccctgctcggcggcgcgcgcggcggaggaatg

SEQ ID NO: 16499 - RNA, 671 nt, Homo sapiens
  source 1..671: mol_type = other RNA
gtgagtctctaagaaaagaggaagtgcagcatatcctgttcaaaagataaacataagcagtttggaaactagtagttacagtgtgggatctgaggaatagaaggagagaaaccaattcaaaccttcctacttaagcagcagaccagcagaactccttcgattacaatacaaactcacttcagcactgctccagagtgtgcagggatgtcgcccacagtcaatggggctagaaactcgggagggggacacctggcaagctgtccttttccttcctggggtctcacgtgtaggagagatacagcgtacctctcagctgcatttctcgatctcctctaagcatgtggatccatccttcttcagcctgatctgcggccctccttggactggacctgagtcgctgaggtcctccaggagcctccagatcacctgcggcgttgttgtctccccagcaatcctggctttgagaatgactgtgcttcttgagtaacaggaagggcatctctgtgatcaatggtataacacttccccatgtctggtttagcactttttgagatctagtgctaacctaggtctagcagttaacctgtttgcttattgactccttctttccagattccaaattgccggaaatataatgagtgtctcagaaataactgcttgaggcattccca

SEQ ID NO: 16500 - RNA, 696 nt, Homo sapiens
  source 1..696: mol_type = other RNA
gtgagtctctaagaaaagaggaagtgcagcatatcctgttcaaaagataaacataagcagtttggaaactagtagttacagtgtgggatctgaggaatagaaggagagaaaccaattcaaaccttcctacttaagcagcagaccagcagaactccttcgattacaatacaaactcacttcagcactgctccagagtgtgcagggatgtcgcccacagtcaatggggctagaaactcgggagggggacacctggcaagctgtccttttccttcctggggtctcacgtgtaggagagatacagcgtacctctcagctgcatttctcgatctcctctaagcatgtggatccatccttcttcagcctgatctgcggccctccttggactggacctgagtcgctgaggtcctccaggagcctccagatcacctgcggcgttgttgtctcctgaatgaactacagtcgtcatatgacacagcaatctcactcccaggtatttaaccttcttttcacagtgcgaggatatataagaaagtcagcagtctgcatggaaaactgggcatggatcgtacccagctggtatccttatcttcaactcccagcctccagaacctcatcttttttttctcatgctgtcacaatctctttgctgggaatttcctctcctcattgagttgtcactcatttatattctctgat

SEQ ID NO: 16501 - RNA, 42 nt, Homo sapiens
  source 1..42: mol_type = other RNA
gtgcatggctgtatatataacagcatccactcaataccatct

SEQ ID NO: 16502 - RNA, 2764 nt, Homo sapiens
  source 1..2764: mol_type = other RNA
gtgcattgctgttgcattgctgagggagatttgttcatgggagaagcaaccctgaggaaaatgcgctgccgccaggagatccggcgaggagtgacagaggttcctcccacacttagggactcattgctgcaggtagatgaggtcctttttctcccttctccatcactgatttcattttcatactgtggggacagtctacctgaattctggtaaaagcttttcaggaaagagggggcagtgaaggaaggggcagagaaggaagtgtgaagacttggaagactggaggaagaattactctccttgtacatgcgtcgaactgacgaaagattgctgcactgttcactggagctctgcctcagcagaggggaacgcacaccctgagccctcccatcctgcaaattcagctttctctttgtgcttgaaggtgggtggctgaacgtgtgtgcccgtcttcgaaactgcggggagtcggaatcctcttcgggaaacgtttgccaagctgaggacggtggggacgctggcggtgtccctggtggagaatcccctggtgagtagtccttctctgaagcaagactgttggaccgttcaaaactgtccacacttccaagccgacctctcattctgttagctccccttgagaagatattttccagggagctagttaaggatctcttagctttatttttcagaatgtcaagtttgaaccttccactgcttgttgcattttctgggattgtactatttgaaatagtagaagggccttccccgatgtgcacgtgtgtcttctgcttggcttcacacagctgcctcaggtgtaaaatcacaagttcattttcttcctggtcactgactggcttcattttctgaactctttcaaagatgtcagcttgctcattatctgtcagtgatgagagatgcctctgtatcaccagcttggctcttggtgggtagagaccttcaatcctttcacagagcttatgcaaagagtgcatcgggcaggcctcacacagtttaatctgcgtcttggcactctgcagggcagccgccgtactgaaggcctgtttcagagtcagcattacctcatcaaccagagattcgctggcacactggaatacataacaaatatactggctaagtccaggctctggagactcccggcagataaagccaaagtgatccacatgctttataccctgagaacaagaggagatatctttaaaattcttttctagcacaactgatttagtgtctggactgataaggttaatctcaaatcgcccaacctggaagagcatggtcctgttcttctccgagtccgagggctggacgtgactgggtgcgctcgcgtgtctccgtcgcggctgggatttctggctgccctcgtgaactctccgttgcacgccggtgacactgctgcaccgagaccgaaactcctgctgctcatcaaagccagaatcttccaaaatccgctcagggaagcagacccgagagctggtcagggcaggctggctggccccggcaggtaagccaaggtgggtgtcggtgccgtcagcctcctccggcaggcagtctccgggggacccgggcaccaccacctccaagtcagccaggtcctctcctgggtccggaccgcgctgctccccttggatcttcaggcgctgctgttcgtgcaggctgaacttctccatgcagtcatcgatgaggcttgagggggccttcttgtgggtcacggtcacctttccacagtacaggacttcgaacttctgagagttgtaaaaggcgtcctcattatctttgctgggtttggcatcctctttcatggccgctttagataattgccttatgctgctaataacatcaggaacctggctggggtctgtggcgcggaaaacgtggcaggccatctgcgactcggggtcgtcgggctgcgccttgatcaggtaggcaaagtaggtgaggtcgtggctgttgtggatgaagcgcgagatatgctgcgccttgtgctcgaagatgaataccgccgggttgggctgcgtggccgacggactagtgccccccgaggccccagcgcccggcgcggggacgcaacgcaggaagggcgcgctgagcaccaggatcacctctcgggccgccggcgccccgcagccgcccgcctcgggcttctggctgcgcctgcggatctcggccatgagccagggcagcataggcagcgtggtcctgtggtccaggcacgaccccccaacgtaccacagccggaaccgcttatcgcttggcttcccggggccgggctgagctgagacgcccggctcgggctccagggggtgcgggaacggctcatcctgaatgcagctgggcggctccataactctcgcctcaccagggcaccgcggaggccggccgggcgcaccgcgccccccactcccgcgcagaaggcgccgccgaaactgtgccaactgccgcaccgggctcccgcgcctgcctgggagcggcgcgaccccgaactccgcgcttcagcagccctgccccatgcagcacttccacgggcgcggctcggaggctccggcggcgggcaccgaggcaagcgcccggcaggcgagggcgggttaaatgggcatcctcctccttgggctggcgcctcgggcaggacctccccttcctccgtcgcgggtttgcagggtcagaggaccacgccgagggtccccgcggccgccggctccagcgctgcagccccgctgcggccgccgcgctcgcctggggcagacac

SEQ ID NO: 16503 - RNA, 2599 nt, Homo sapiens
  source 1..2599: mol_type = other RNA
gtgcattgctgttgcattgctgagggagatttgttcatgggagaagcaaccctgaggaaaatgcgctgccgccaggagatccggcgaggagtgacagaggttcctcccacacttagggactcattgctgcaggtagatgaggtcctttttctcccttctccatcactgcactgttcactggagctctgcctcagcagaggggaacgcacaccctgagccctcccatcctgcaaattcagctttctctttgtgcttgaaggtgggtggctgaacgtgtgtgcccgtcttcgaaactgcggggagtcggaatcctcttcgggaaacgtttgccaagctgaggacggtggggacgctggcggtgtccctggtggagaatcccctggtgagtagtccttctctgaagcaagactgttggaccgttcaaaactgtccacacttccaagccgacctctcattctgttagctccccttgagaagatattttccagggagctagttaaggatctcttagctttatttttcagaatgtcaagtttgaaccttccactgcttgttgcattttctgggattgtactatttgaaatagtagaagggccttccccgatgtgcacgtgtgtcttctgcttggcttcacacagctgcctcaggtgtaaaatcacaagttcattttcttcctggtcactgactggcttcattttctgaactctttcaaagatgtcagcttgctcattatctgtcagtgatgagagatgcctctgtatcaccagcttggctcttggtgggtagagaccttcaatcctttcacagagcttatgcaaagagtgcatcgggcaggcctcacacagtttaatctgcgtcttggcactctgcagggcagccgccgtactgaaggcctgtttcagagtcagcattacctcatcaaccagagattcgctggcacactggaatacataacaaatatactggctaagtccaggctctggagactcccggcagataaagccaaagtgatccacatgctttataccctgagaacaagaggagatatctttaaaattcttttctagcacaactgatttagtgtctggactgataaggttaatctcaaatcgcccaacctggaagagcatggtcctgttcttctccgagtccgagggctggacgtgactgggtgcgctcgcgtgtctccgtcgcggctgggatttctggctgccctcgtgaactctccgttgcacgccggtgacactgctgcaccgagaccgaaactcctgctgctcatcaaagccagaatcttccaaaatccgctcagggaagcagacccgagagctggtcagggcaggctggctggccccggcaggtaagccaaggtgggtgtcggtgccgtcagcctcctccggcaggcagtctccgggggacccgggcaccaccacctccaagtcagccaggtcctctcctgggtccggaccgcgctgctccccttggatcttcaggcgctgctgttcgtgcaggctgaacttctccatgcagtcatcgatgaggcttgagggggccttcttgtgggtcacggtcacctttccacagtacaggacttcgaacttctgagagttgtaaaaggcgtcctcattatctttgctgggtttggcatcctctttcatggccgctttagataattgccttatgctgctaataacatcaggaacctggctggggtctgtggcgcggaaaacgtggcaggccatctgcgactcggggtcgtcgggctgcgccttgatcaggtaggcaaagtaggtgaggtcgtggctgttgtggatgaagcgcgagatatgctgcgccttgtgctcgaagatgaataccgccgggttgggctgcgtggccgacggactagtgccccccgaggccccagcgcccggcgcggggacgcaacgcaggaagggcgcgctgagcaccaggatcacctctcgggccgccggcgccccgcagccgcccgcctcgggcttctggctgcgcctgcggatctcggccatgagccagggcagcataggcagcgtggtcctgtggtccaggcacgaccccccaacgtaccacagccggaaccgcttatcgcttggcttcccggggccgggctgagctgagacgcccggctcgggctccagggggtgcgggaacggctcatcctgaatgcagctgggcggctccataactctcgcctcaccagggcaccgcggaggccggccgggcgcaccgcgccccccactcccgcgcagaaggcgccgccgaaactgtgccaactgccgcaccgggctcccgcgcctgcctgggagcggcgcgaccccgaactccgcgcttcagcagccctgccccatgcagcacttccacgggcgcggctcggaggctccggcggcgggcaccgaggcaagcgcccggcaggcgagggcgggttaaatgggcatcctcctccttgggctggcgcctcgggcaggacctccccttcctccgtcgcgggtttgcagggtcagaggaccacgccgagggtccccgcggccgccggctccagcgctgcagccccgctgcggccgccgcgctcgcctggggcagacac

SEQ ID NO: 16504 - RNA, 1802 nt, Homo sapiens
  source 1..1802: mol_type = other RNA
gtgcattgctgttgcattgctgagggagatttgttcatgggagaagcaaccctgaggaaaatgcgctgccgccaggagatccggcgaggagtgacagaggttcctcccacacttagggactcattgctgcaggtagatgaggtcctttttctcccttctccatcactgcactgttcactggagctctgcctcagcagaggggaacgcacaccctgagccctcccatcctgcaaattcagctttctctttgtgcttgaaggtgggtggctgaacgtgtgtgcccgtcttcgaaactgcggggagtcggaatcctcttcgggaaacgtttgccaagctgaggacggtggggacgctggcggtgtccctggtggagaatcccctggtgagtagtccttctctgaagcaagactgttggaccgttcaaaactgtccacacttccaagccgacctctcattctgttagctccccttgagaagatattttccagggagctagttaaggatctcttagctttatttttcagaatgtcaagtttgaaccttccactgcttgttgcattttctgggattgtactatttgaaatagtagaagggccttccccgatgtgcacgtgtgtcttctgcttggcttcacacagctgcctcaggtgtaaaatcacaagttcattttcttcctggtcactgactggcttcattttctgaactctttcaaagatgtcagcttgctcattatctgtcagtgatgagagatgcctctgtatcaccagcttggctcttggtgggtagagaccttcaatcctttcacagagcttatgcaaagagtgcatcgggcaggcctcacacagtttaatctgcgtcttggcactctgcagggcagccgccgtactgaaggcctgtttcagagtcagcattacctcatcaaccagagattcgctggcacactggaatacataacaaatatactggctaagtccaggctctggagactcccggcagataaagccaaagtgatccacatgctttataccctgagaacaagaggagatatctttaaaattcttttctagcacaactgatttagtgtctggactgataaggttaatctcaaatcgcccaacctggaagagcatggtcctgttcttctccgagtccgagggctggacgtgactgggtgcgctcgcgtgtctccgtcgcggctgggatttctggctgccctcgtgaactctccgttgcacgccggtgacactgctgcaccgagaccgaaactcctgctgctcatcaaagccagaatcttccaaaatccgctcagggaagcagacccgagagctggtcagggcaggctggctggccccggcaggtaagccaaggtgggtgtcggtgccgtcagcctcctccggcaggcagtctccgggggacccgggcaccaccacctccaagtcagccaggtcctctcctgggtccggaccgcgctgctccccttggatcttcaggcgctgctgttcgtgcaggctgaacttctccatgcagtcatcgatgaggcttgagggggccttcttgtgggtcacggtcacctttccacagtacaggacttcgaacttctgagagttgtaaaaggcgtcctcattatctttgctgggtttggcatcctctttcatggccgctttagataattgccttatgctgctaataacatcaggaacctttgatcaggaagccagctggaaactggaggtggtcacgaagagcaatgattttgccaaactggtgtagtcctcagtattagctctaagttctctctttct

SEQ ID NO: 16505 - RNA, 1691 nt, Homo sapiens
  source 1..1691: mol_type = other RNA
gtgcattgctgttgcattgctgagggagatttgttcatgggagaagcaaccctgaggaaaatgcgctgccgccaggagatccggcgaggagtgacagaggttcctcccacacttagggactcattgctgcaggtagatgaggtcctttttctcccttctccatcactgcactgttcactggagctctgcctcagcagaggggaacgcacaccctgagccctcccatcctgcaaattcagctttctctttgtgcttgaaggtgggtggctgaacgtgtgtgcccgtcttcgaaactgcggggagtcggaatcctcttcgggaaacgtttgccaagctgaggacggtggggacgctggcggtgtccctggtggagaatcccctggtgagtagtccttctctgaagcaagactgttggaccgttcaaaactgtccacacttccaagccgacctctcattctgttagctccccttgagaagatattttccagggagctagttaaggatctcttagctttatttttcagaatgtcaagtttgaaccttccactgcttgttgcattttctgggattgtactatttgaaatagtctgaactctttcaaagatgtcagcttgctcattatctgtcagtgatgagagatgcctctgtatcaccagcttggctcttggtgggtagagaccttcaatcctttcacagagcttatgcaaagagtgcatcgggcaggcctcacacagtttaatctgcgtcttggcactctgcagggcagccgccgtactgaaggcctgtttcagagtcagcattacctcatcaaccagagattcgctggcacactggaatacataacaaatatactggctaagtccaggctctggagactcccggcagataaagccaaagtgatccacatgctttataccctgagaacaagaggagatatctttaaaattcttttctagcacaactgatttagtgtctggactgataaggttaatctcaaatcgcccaacctggaagagcatggtcctgttcttctccgagtccgagggctggacgtgactgggtgcgctcgcgtgtctccgtcgcggctgggatttctggctgccctcgtgaactctccgttgcacgccggtgacactgctgcaccgagaccgaaactcctgctgctcatcaaagccagaatcttccaaaatccgctcagggaagcagacccgagagctggtcagggcaggctggctggccccggcaggtaagccaaggtgggtgtcggtgccgtcagcctcctccggcaggcagtctccgggggacccgggcaccaccacctccaagtcagccaggtcctctcctgggtccggaccgcgctgctccccttggatcttcaggcgctgctgttcgtgcaggctgaacttctccatgcagtcatcgatgaggcttgagggggccttcttgtgggtcacggtcacctttccacagtacaggacttcgaacttctgagagttgtaaaaggcgtcctcattatctttgctgggtttggcatcctctttcatggccgctttagataattgccttatgctgctaataacatcaggaacctttgatcaggaagccagctggaaactggaggtggtcacgaagagcaatgattttgccaaactggtgtagtcctcagtattagctctaagttctctctttct

SEQ ID NO: 16506 - RNA, 3689 nt, Homo sapiens
  source 1..3689: mol_type = other RNA
gtgcattgctgttgcattgctgagggagatttgttcatgggagaagcaaccctgaggaaaatgcgctgccgccaggagatccggcgaggagtgacagaggttcctcccacacttagggactcattgctgcaggtagatgaggtcctttttctcccttctccatcacttgattctgaagcagtgtcttgtctgatttcattttcatactgtggggacagtctacctgaattctggtaaaagcttttcaggaaagagggggcagtgaaggaaggggcagagaaggaagtgtgaagacttggaagactggaggaagaattactctccttgtacatgcgtcgaactgacgaaagattgctgcactgttcactggagctctgcctcagcagaggggaacgcacaccctgagccctcccatcctgcaaattcagctttctctttgtgcttgaaggtgggtggctgaacgtgtgtgcccgtcttcgaaactgcggggagtcggaatcctcttcgggaaacgtttgccaagctgaggacggtggggacgctggcggtgtccctggtggagaatcccctggtgagtagtcccttgagaagatattttccagggagctagttaaggatctcttagctttatttttcagaatgtcaagtttgaaccttccactgcttgttgcattttctgggattgtactatttgaaatagtagaagggccttccccgatgtgcacgtgtgtcttctgcttggcttcacacagctgcctcaggtgtaaaatcacaagttcattttcttcctggtcactgactggcttcattttctgaactctttcaaagatgtcagcttgctcattatctgtcagtgatgagagatgcctctgtatcaccagcttggctcttggtgggtagagaccttcaatcctttcacagagcttatgcaaagagtgcatcgggcaggcctcacacagtttaatctgcgtcttggcactctgcagggcagccgccgtactgaaggcctgtttcagagtcagcattacctcatcaaccagagattcgctggcacactggaatacataacaaatatactggctaagtccaggctctggagactcccggcagataaagccaaagtgatccacatgctttataccctgagaacaagaggagatatctttaaaattcttttctagcacaactgatttagtgtctggactgataaggttaatctcaaatcgcccaacctggaagagcatggtcctgttcttctccgagtccgagggctggacgtgactgggtgcgctcgcgtgtctccgtcgcggctgggatttctggctgccctcgtgaactctccgttgcacgccggtgacactgctgcaccgagaccgaaactcctgctgctcatcaaagccagaatcttccaaaatccgctcagggaagcagacccgagagctggtcagggcaggctggctggccccggcaggtaagccaaggtgggtgtcggtgccgtcagcctcctccggcaggcagtctccgggggacccgggcaccaccacctccaagtcagccaggtcctctcctgggtccggaccgcgctgctccccttggatcttcaggcgctgctgttcgtgcaggctgaacttctccatgcagtcatcgatgaggcttgagggggccttcttgtgggtcacggtcacctttccacagtacaggacttcgaacttctgagagttgtaaaaggcgtcctcattatctttgctgggtttggcatcctctttcatggccgctttagataattgccttatgctgctaataacatcaggaacctggctggggtctgtggcgcggaaaacgtggcaggccatctgcgactcggggtcgtcgggctgcgccttgatcaggtaggcaaagtaggtgaggtcgtggctgttgtggatgaagcgcgagatatgctgcgccttgtgctcgaagatgaataccgccgggttgggctgcgtggccgacggactagtgccccccgaggccccagcgcccggcgcggggacgcaacgcaggaagggcgcgctgagcaccaggatcacctctcgggccgccggcgccccgcagccgcccgcctcgggcttctggctgcgcctgcggatctcggccatgagccagggcagcataggcagcgtggtcctgtggtccaggcacgaccccccaacgtaccacagccggaaccgcttatcgcttggcttcccggggccgggctgagctgagacgcccggctcgggctccagggggtgcgggaacggctcatcctgaatgcagctgggcggctccataactctcgcctcaccagggcaccgcggaggccggccgggcgcaccgcgccccccactcccgcgcagaaggcgccgccgaaactgtgccaactgccgcaccgggctcccgcgcctgcctgggagcggcgcgaccccgaactccgcgcttcagcagccctgccccatgcagcacttccacgggcgcggctcggaggctccggcggcgggcaccgaggcaagcgcccggcaggcgagggcgggttaaatgggcatcctcctccttgggctggcgcctcgggcaggacctccccttcctccgtcgcgggtttgcagggtcagaggaccacgccgagggtccccgcggccgccggctccagcgctgcagccccgctgcggccgccgcgctcgcctggggcagacactgggtggctgggcggggaatggggctgtgggcgggagggggtgacttggggcggagctgactcctaccagggtgaccggctgtcacctggaaggtcggggctgcagggctgcggcgcggtcagtcctcaggaaaggctccggcaactactccagtggaaaataacaaaaacaaaacgtggcctcgcgggggccgctcctcctcccgccgcagctgcagcccagctcgctgctcctcctcctgccgttcccgtccctccctcgctccttccttccttccttccaggctgcttctttaatcgggctgctactccgcctcccgtccggcgggcggagagcgtcgcctgcaaaagcttatccgtgaagccgcctctccgcctcttcgcctcttccttcgacccccgcccttggggctgcagctcagagcctggcgcgggcactgcccggacccacttggcctctcttgagtcgccgcgatctccgtctcctcccgggcgtctctgctgccccctagagagggggccactcgcagtggagaactgggatttttttttaacagtatttgcttggtttcagttccttctaaagcctacacattaatttctgaattatctttcctaataatctcaaaaaacgctcgtgttttcaatcacaatattataaattccagttccaaatttcactttaaaacataatatcgacagcttgaatcttcctagttattaaagcagccaacttcttaaaatatggaaaagttatgttttatttatgttatatccccagttgagagctaatgtagagatttcttgttcttttatatatatgtggtaatacatatttccaaagaactaaaaaaaagtttggaataatttgatcattgtaattttaagacaggtagacaagtattctccctttttactcataccgaatgataattaagaattgggtaagaagtaaagacaaaataaataagaaaga

SEQ ID NO: 16507 - RNA, 2476 nt, Homo sapiens
  source 1..2476: mol_type = other RNA
gtgcattgctgttgcattgctgagggagatttgttcatgggagaagcaaccctgaggaaaatgcgctgccgccaggagatccggcgaggagtgacagaggttcctcccacacttagggactcattgctgcaggtagatgaggtcctttttctcccttctccatcacttgattctgaagcagtgtcttgtctgatttcattttcatactgtggggacagtctacctgaattctggtaaaagcttttcaggaaagagggggcagtgaaggaaggggcagagaaggaagtgtgaagacttggaagactggaggaagaattactctccttgtacatgcgtcgaactgacgaaagattgctgcactgttcactggagctctgcctcagcagaggggaacgcacaccctgagccctcccatcctgcaaattcagctttctctttgtgcttgaaggtgggtggctgaacgtgtgtgcccgtcttcgaaactgcggggagtcggaatcctcttcgggaaacgtttgccaagctgaggacggtggggacgctggcggtgtccctggtggagaatcccctggtgagtagtccttctctgaagcaagactgttggaccgttcaaaactgtccacacttccaagccgacctctcattctgttagctccccttgagaagatattttccagggagctagttaaggatctcttagctttatttttcagaatgtcaagtttgaaccttccactgcttgttgcattttctgggattgtactatttgaaatagtagaagggccttccccgatgtgcacgtgtgtcttctgcttggcttcacacagctgcctcaggtgtaaaatcacaagttcattttcttcctggtcactgactggcttcattttctgaactctttcaaagatgtcagcttgctcattatctgtcagtgatgagagatgcctctgtatcaccagcttggctcttggtgggtagagaccttcaatcctttcacagagcttatgcaaagagtgcatcgggcaggcctcacacagtttaatctgcgtcttggcactctgcagggcagccgccgtactgaaggcctgtttcagagtcagcattacctcatcaaccagagattcgctggcacactggaatacataacaaatatactggctaagtccaggctctggagactcccggcagataaagccaaagtgatccacatgctttataccctgagaacaagaggagatatctttaaaattcttttctagcacaactgatttagtgtctggactgataaggttaatctcaaatcgcccaacctggaagagcatggtcctgttcttctccgagtccgagggctggacgtgactgggtgcgctcgcgtgtctccgtcgcggctgggatttctggctgccctcgtgaactctccgttgcacgccggtgacactgctgcaccgagaccgaaactcctgctgctcatcaaagccagaatcttccaaaatccgctcagggaagcagacccgagagctggtcagggcaggctggctggccccggcaggtaagccaaggtgggtgtcggtgccgtcagcctcctccggcaggcagtctccgggggacccgggcaccaccacctccaagtcagccaggtcctctcctgggtccggaccgcgctgctccccttggatcttcaggcgctgctgttcgtgcaggctgaacttctccatgcagtcatcgatgaggcttgagggggccttcttgtgggtcacggtcacctttccacagtacaggacttcgaacttctgagagttgtaaaaggcgtcctcattatctttgctgggtttggcatcctctttcatggccgctttagataattgccttatgctgctaataacatcaggaacacaaggtgtctgaacatcttccatcccctgtcaaaatcagaggaagctgtgaagcctgccagccatcaggcccgggttaatgagttccacagtccagtttcacagtatctctggcatttgcagtcatggggaaagaacatgcagcccccgtgctcctgggcccctctctcaagagtctgtttcaggcatgcagggctaaaataaaccaaaccagcagactgaactgcctttcacccatggataaagacctactcctgtccatggccaggtaccaggagatcctgggtcaatgcatttttaattccaccggatcctctacttcacaacatgactttctttatttttaggggaaaagtgtgtggggtttttgcaggggagaaaggattaagataattattagttctagtttcgcagctagcaacaaaatcacttgctaacaactagtttttcattattactaaacaaaatattttaattgtaggctctattcatattgcttaaagaaattacattctaaatgttttgagatattcttgtatgttaacaggtagttacaaaatgtattatttttgatctagcaaatacct

SEQ ID NO: 16508 - RNA, 2789 nt, Homo sapiens
  source 1..2789: mol_type = other RNA
gtgcattgctgttgcattgctgagggagatttgttcatgggagaagcaaccctgaggaaaatgcgctgccgccaggagatccggcgaggagtgacagaggttcctcccacacttagggactcattgctgcaggtagatgaggtcctttttctcccttctccatcacttgattctgaagcagtgtcttgtctgatttcattttcatactgtggggacagtctacctgaattctggtaaaagcttttcaggaaagagggggcagtgaaggaaggggcagagaaggaagtgtgaagacttggaagactggaggaagaattactctccttgtacatgcgtcgaactgacgaaagattgctgcactgttcactggagctctgcctcagcagaggggaacgcacaccctgagccctcccatcctgcaaattcagctttctctttgtgcttgaaggtgggtggctgaacgtgtgtgcccgtcttcgaaactgcggggagtcggaatcctcttcgggaaacgtttgccaagctgaggacggtggggacgctggcggtgtccctggtggagaatcccctggtgagtagtccttctctgaagcaagactgttggaccgttcaaaactgtccacacttccaagccgacctctcattctgttagctccccttgagaagatattttccagggagctagttaaggatctcttagctttatttttcagaatgtcaagtttgaaccttccactgcttgttgcattttctgggattgtactatttgaaatagtagaagggccttccccgatgtgcacgtgtgtcttctgcttggcttcacacagctgcctcaggtgtaaaatcacaagttcattttcttcctggtcactgactggcttcattttctgaactctttcaaagatgtcagcttgctcattatctgtcagtgatgagagatgcctctgtatcaccagcttggctcttggtgggtagagaccttcaatcctttcacagagcttatgcaaagagtgcatcgggcaggcctcacacagtttaatctgcgtcttggcactctgcagggcagccgccgtactgaaggcctgtttcagagtcagcattacctcatcaaccagagattcgctggcacactggaatacataacaaatatactggctaagtccaggctctggagactcccggcagataaagccaaagtgatccacatgctttataccctgagaacaagaggagatatctttaaaattcttttctagcacaactgatttagtgtctggactgataaggttaatctcaaatcgcccaacctggaagagcatggtcctgttcttctccgagtccgagggctggacgtgactgggtgcgctcgcgtgtctccgtcgcggctgggatttctggctgccctcgtgaactctccgttgcacgccggtgacactgctgcaccgagaccgaaactcctgctgctcatcaaagccagaatcttccaaaatccgctcagggaagcagacccgagagctggtcagggcaggctggctggccccggcaggtaagccaaggtgggtgtcggtgccgtcagcctcctccggcaggcagtctccgggggacccgggcaccaccacctccaagtcagccaggtcctctcctgggtccggaccgcgctgctccccttggatcttcaggcgctgctgttcgtgcaggctgaacttctccatgcagtcatcgatgaggcttgagggggccttcttgtgggtcacggtcacctttccacagtacaggacttcgaacttctgagagttgtaaaaggcgtcctcattatctttgctgggtttggcatcctctttcatggccgctttagataattgccttatgctgctaataacatcaggaacctggctggggtctgtggcgcggaaaacgtggcaggccatctgcgactcggggtcgtcgggctgcgccttgatcaggtaggcaaagtaggtgaggtcgtggctgttgtggatgaagcgcgagatatgctgcgccttgtgctcgaagatgaataccgccgggttgggctgcgtggccgacggactagtgccccccgaggccccagcgcccggcgcggggacgcaacgcaggaagggcgcgctgagcaccaggatcacctctcgggccgccggcgccccgcagccgcccgcctcgggcttctggctgcgcctgcggatctcggccatgagccagggcagcataggcagcgtggtcctgtggtccaggcacgaccccccaacgtaccacagccggaaccgcttatcgcttggcttcccggggccgggctgagctgagacgcccggctcgggctccagggggtgcgggaacggctcatcctgaatgcagctgggcggctccataactctcgcctcaccagggcaccgcggaggccggccgggcgcaccgcgccccccactcccgcgcagaaggcgccgccgaaactgtgccaactgccgcaccgggctcccgcgcctgcctgggagcggcgcgaccccgaactccgcgcttcagcagccctgccccatgcagcacttccacgggcgcggctcggaggctccggcggcgggcaccgaggcaagcgcccggcaggcgagggcgggttaaatgggcatcctcctccttgggctggcgcctcgggcaggacctccccttcctccgtcgcgggtttgcagggtcagaggaccacgccgagggtccccgcggccgccggctccagcgctgcagccccgctgcggccgccgcgctcgcctggggcagacact

SEQ ID NO: 16509 - RNA, 1991 nt, Homo sapiens
  source 1..1991: mol_type = other RNA
gtgcattgctgttgcattgctgagggagatttgttcatgggagaagcaaccctgaggaaaatgcgctgccgccaggagatccggcgaggagtgacagaggttcctcccacacttagggactcattgctgcaggtagatgaggtcctttttctcccttctccatcacttgattctgaagcagtgtcttgtctgatttcattttcatactgtggggacagtctacctgaattctggtaaaagcttttcaggaaagagggggcagtgaaggaaggggcagagaaggaagtgtgaagacttggaagactggaggaagaattactctccttgtacatgcgtcgaactgacgaaagattgctgcactgttcactggagctctgcctcagcagaggggaacgcacaccctgagccctcccatcctgcaaattcagctttctctttgtgcttgaaggtgggtggctgaacgtgtgtgcccgtcttcgaaactgcggggagtcggaatcctcttcgggaaacgtttgccaagctgaggacggtggggacgctggcggtgtccctggtggagaatcccctggtgagtagtccttctctgaagcaagactgttggaccgttcaaaactgtccacacttccaagccgacctctcattctgttagctccccttgagaagatattttccagggagctagttaaggatctcttagctttatttttcagaatgtcaagtttgaaccttccactgcttgttgcattttctgggattgtactatttgaaatagtagaagggccttccccgatgtgcacgtgtgtcttctgcttggcttcacacagctgcctcaggtgtaaaatcacaagttcattttcttcctggtcactgactggcttcattttctgaactctttcaaagatgtcagcttgctcattatctgtcagtgatgagagatgcctctgtatcaccagcttggctcttggtgggtagagaccttcaatcctttcacagagcttatgcaaagagtgcatcgggcaggcctcacacagtttaatctgcgtcttggcactctgcagggcagccgccgtactgaaggcctgtttcagagtcagcattacctcatcaaccagagattcgctggcacactggaatacataacaaatatactggctaagtccaggctctggagactcccggcagataaagccaaagtgatccacatgctttataccctgagaacaagaggagatatctttaaaattcttttctagcacaactgatttagtgtctggactgataaggttaatctcaaatcgcccaacctggaagagcatggtcctgttcttctccgagtccgagggctggacgtgactgggtgcgctcgcgtgtctccgtcgcggctgggatttctggctgccctcgtgaactctccgttgcacgccggtgacactgctgcaccgagaccgaaactcctgctgctcatcaaagccagaatcttccaaaatccgctcagggaagcagacccgagagctggtcagggcaggctggctggccccggcaggtaagccaaggtgggtgtcggtgccgtcagcctcctccggcaggcagtctccgggggacccgggcaccaccacctccaagtcagccaggtcctctcctgggtccggaccgcgctgctccccttggatcttcaggcgctgctgttcgtgcaggctgaacttctccatgcagtcatcgatgaggcttgagggggccttcttgtgggtcacggtcacctttccacagtacaggacttcgaacttctgagagttgtaaaaggcgtcctcattatctttgctgggtttggcatcctctttcatggccgctttagataattgccttatgctgctaataacatcaggaacctttgatcaggaagccagctggaaactggaggtggtcacgaagagcaatgattttgccaaactggtgtagtcctcagtattagctctaagttctctctttct

SEQ ID NO: 16510 - RNA, 3653 nt, Homo sapiens
  source 1..3653: mol_type = other RNA
gtgcattgctgttgcattgctgagggagatttgttcatgggagaagcaaccctgaggaaaatgcgctgccgccaggagatccggcgaggagtgacagaggttcctcccacacttagggactcattgctgcaggtagatgaggtcctttttctcccttctccatcacttgattctgaagcagtgtcttgtctgatttcattttcatactgtggggacagtctacctgaattctggtaaaagcttttcaggaaagagggggcagtgaaggaaggggcagagaaggaagtgtgaagacttggaagactggaggaagaattactctccttgtacatgcgtcgaactgacgaaagattgctgcactgttcactggagctctgcctcagcagaggggaacgcacaccctgagccctcccatcctgcaaattcagctttctctttgtgcttgaaggtgggtggctgaacgtgtgtgcccgtcttcgaaactgcggggagtcggaatcctcttcgggaaacgtttgccaagctgaggacggtggggacgctggcggtgtccctggtggagaatcccctggtgagtagtccttctctgaagcaagactgttggaccgttcaaaactgtccacacttccaagccgacctctcattctgttagctccccttgagaagatattttccagggagctagttaaggatctcttagctttatttttcagaatgtcaagtttgaaccttccactgcttgttgcattttctgggattgtactatttgaaatagtctgaactctttcaaagatgtcagcttgctcattatctgtcagtgatgagagatgcctctgtatcaccagcttggctcttggtgggtagagaccttcaatcctttcacagagcttatgcaaagagtgcatcgggcaggcctcacacagtttaatctgcgtcttggcactctgcagggcagccgccgtactgaaggcctgtttcagagtcagcattacctcatcaaccagagattcgctggcacactggaatacataacaaatatactggctaagtccaggctctggagactcccggcagataaagccaaagtgatccacatgctttataccctgagaacaagaggagatatctttaaaattcttttctagcacaactgatttagtgtctggactgataaggttaatctcaaatcgcccaacctggaagagcatggtcctgttcttctccgagtccgagggctggacgtgactgggtgcgctcgcgtgtctccgtcgcggctgggatttctggctgccctcgtgaactctccgttgcacgccggtgacactgctgcaccgagaccgaaactcctgctgctcatcaaagccagaatcttccaaaatccgctcagggaagcagacccgagagctggtcagggcaggctggctggccccggcaggtaagccaaggtgggtgtcggtgccgtcagcctcctccggcaggcagtctccgggggacccgggcaccaccacctccaagtcagccaggtcctctcctgggtccggaccgcgctgctccccttggatcttcaggcgctgctgttcgtgcaggctgaacttctccatgcagtcatcgatgaggcttgagggggccttcttgtgggtcacggtcacctttccacagtacaggacttcgaacttctgagagttgtaaaaggcgtcctcattatctttgctgggtttggcatcctctttcatggccgctttagataattgccttatgctgctaataacatcaggaacctggctggggtctgtggcgcggaaaacgtggcaggccatctgcgactcggggtcgtcgggctgcgccttgatcaggtaggcaaagtaggtgaggtcgtggctgttgtggatgaagcgcgagatatgctgcgccttgtgctcgaagatgaataccgccgggttgggctgcgtggccgacggactagtgccccccgaggccccagcgcccggcgcggggacgcaacgcaggaagggcgcgctgagcaccaggatcacctctcgggccgccggcgccccgcagccgcccgcctcgggcttctggctgcgcctgcggatctcggccatgagccagggcagcataggcagcgtggtcctgtggtccaggcacgaccccccaacgtaccacagccggaaccgcttatcgcttggcttcccggggccgggctgagctgagacgcccggctcgggctccagggggtgcgggaacggctcatcctgaatgcagctgggcggctccataactctcgcctcaccagggcaccgcggaggccggccgggcgcaccgcgccccccactcccgcgcagaaggcgccgccgaaactgtgccaactgccgcaccgggctcccgcgcctgcctgggagcggcgcgaccccgaactccgcgcttcagcagccctgccccatgcagcacttccacgggcgcggctcggaggctccggcggcgggcaccgaggcaagcgcccggcaggcgagggcgggttaaatgggcatcctcctccttgggctggcgcctcgggcaggacctccccttcctccgtcgcgggtttgcagggtcagaggaccacgccgagggtccccgcggccgccggctccagcgctgcagccccgctgcggccgccgcgctcgcctggggcagacactgggtggctgggcggggaatggggctgtgggcgggagggggtgacttggggcggagctgactcctaccagggtgaccggctgtcacctggaaggtcggggctgcagggctgcggcgcggtcagtcctcaggaaaggctccggcaactactccagtggaaaataacaaaaacaaaacgtggcctcgcgggggccgctcctcctcccgccgcagctgcagcccagctcgctgctcctcctcctgccgttcccgtccctccctcgctccttccttccttccttccaggctgcttctttaatcgggctgctactccgcctcccgtccggcgggcggagagcgtcgcctgcaaaagcttatccgtgaagccgcctctccgcctcttcgcctcttccttcgacccccgcccttggggctgcagctcagagcctggcgcgggcactgcccggacccacttggcctctcttgagtcgccgcgatctccgtctcctcccgggcgtctctgctgccccctagagagggggccactcgcagtggagaactgggatttttttttaacagtatttgcttggtttcagttccttctaaagcctacacattaatttctgaattatctttcctaataatctcaaaaaacgctcgtgttttcaatcacaatattataaattccagttccaaatttcactttaaaacataatatcgacagcttgaatcttcctagttattaaagcagccaacttcttaaaatatggaaaagttatgttttatttatgttatatccccagttgagagctaatgtagagatttcttgttcttttatatatatgtggtaatacatatttccaaagaactaaaaaaaagtttggaataatttgatcattgtaattttaagacaggtagacaagtattctccctttttactcataccgaatgataattaagaattgggtaagaagtaaagacaaaataaataagaaaga

SEQ ID NO: 16511 - RNA, 2445 nt, Homo sapiens
  source 1..2445: mol_type = other RNA
gtgccagctgcagtgggggaggtaggtctttgctcttgaggggttcctgatctgtgagccaagccattttttaaactgactgctctttgtagcgggtggataagaggcaaggactaaacagggctaccttaagataacactctaaggatgtcatcatgattcttagggactgtgcatcgcaccttattcagtactcaaagcccaggtatttgccctgcccaggactgctcatggatcataccagttgttcctggggcagagtgatgaggatcttatatcactgggcatagggtcttctgggctgggccttgaaggacagaagcctgctttactctccgctttttgacctagcctccacttcctcactctttgtctgttctgcaagtttgtactcacttctcatctggagcttgccatggctcctgggatcccagcttcctgctctgctgaggaccatggtcggtgttcccccagcagcttccttttaagcagtccctggcccaagctacatgctcagtgaatatccctgcattgactcactgaggccactccggcccagctgcctattgctcctacgctatggccctttagtctcaatggaaattgaaatctggagtgttgggctggccagttatcctctgtccagtgagggccctgtctaactttcttgtctttatttcttttctcagcacaggtttgggctatcacctgagaacattcaggagacagtacaggttcccagatgcaacgactcactcagatttgtcttaacagacccttctactggcaatctcaggtggagcaaaaaggagcgatcattagaaacaaattcattgtggtctcttgattctggccagctactctgcaaagtctggcctcctgcacctcttgggatgaggtggggcctcttgtcaagacaaaagggagcaagggcccctgtagggggaagaagggctgcccaggcctggtgtcagttgttcctggggcagagtgacagggacctcttatcactggccacccagtgtctatggaccttggataccatggcccccaaggtttaaaaaataatggaaaaagccaagatggcaggatttaagcatctcaacatggtcattgccactggagcctctgggctgcatgggcctctggcaggaggagggggtcagggccaggaatcaattataggcaaaggctggctcccttggggctggtgccagggagaaagccagctgcctcatcgcagtgtccaggagaatttatgagttggatcttgggggtgagtggtgaaggttgagctctccaggaagcagactctcagaaggagtttatgaagcaggacgcttaagaggaatgccttgagacaaacacctgtgggaaacggggagggaggcaggatggggcaggggagaggtggagctgtgatgtggcttggctgacaccacagagttgttggaactcagctagctcctcagcgtcatctcatgtggggctctggcagccaggcctctgcatcttacctcctcagtcagaggctactggaacctgaccatcctttaaggactctagaatcaccctgactcctctggttctctcaaagcccacacccaattcttcaccaatccctgtggcctgcatcttacaaacagatccagcctccaagcgtaggtgtcttccttcctccacggcattgtccacgcttccaccacctctcccagagccactgcaacagcctcctgcctcacctccctgcttccactcttggccctctggttgtttctttaccctgaaccacagcatcattttagaatagacatcagaacttgccattcctccacccttactcccatgacttccctgactcacacaggccaagagtcaacgcctcgccactctctcccagctcagccccctccctcctgttcttgggacatgccaggcttgctcccggctcaagatgggtgtacttgcccttttacctgcccactgggctttccccaagacagctacagagcgcatttcctccctgccttcagatccctgttcaaataccatttcctcccagggtccttccctggtcatgctatatgaagttgcaaacccggcccaccccatgatattccctttgaagtttgatgtgtctttggggcaccaaatgtatacaagaatctggagttcaaaagagagctccagactggtgaaaaagatttctgtgtcctggtaatacagatgacattcacacagtgaggatggagaggatcccctagggctgtcttgtccaatctagaagccaccagccacacttggctactgagcactggaaatatggctggtctgcaggggtcatgttgcatgaaagggtaacatgcacagcagattttgaagatttagaaaaaaaaagtaaaatatcccattgataatttttatattgcttacatgttgcaatga

SEQ ID NO: 16512 - RNA, 86 nt, Homo sapiens
  source 1..86: mol_type = other RNA
gtgcgtggtggctcgaggcggggaaaagctgcagcccccagtgcgagatcccagacggttagctggcacagctgcccgcccgcggt

SEQ ID NO: 16513 - RNA, 125 nt, Homo sapiens
  source 1..125: mol_type = other RNA
gtgcgtggtggctcgaggcggggaaaagctgcagcccccagtgcgagatcccagacggttagctggcacagctgcccgcccgcggtagagcccctgctcggcaaccgctccctagcccttctctg

SEQ ID NO: 16514 - RNA, 130 nt, Homo sapiens
  source 1..130: mol_type = other RNA
gtgcgtggtggctcgaggcggggaaaagctgcagcccccagtgcgagatcccagacggttagctggcacagctgcccgcccgcggtagagcccctgctcggcaaccgctccctagcccttctctgctatt

SEQ ID NO: 16515 - RNA, 135 nt, Homo sapiens
  source 1..135: mol_type = other RNA
gtgcgtggtggctcgaggcggggaaaagctgcagcccccagtgcgagatcccagacggttagctggcacagctgcccgcccgcggtagagcccctgctcggcaaccgctccctagcccttctctgctattacgtc

SEQ ID NO: 16516 - RNA, 71 nt, Homo sapiens
  source 1..71: mol_type = other RNA
gtggaccaggatggcaagggctctactgtcctttcaggagagcccttgccatcctggtccactgcatatag

SEQ ID NO: 16517 - RNA, 71 nt, Homo sapiens
  source 1..71: mol_type = other RNA
gtggaccaggatggcaagggctctcctgaaaggacagtagagcccttgccatcctggtccactgcatatag

SEQ ID NO: 16518 - RNA, 3651 nt, Homo sapiens
  source 1..3651: mol_type = other RNA
gtggagtcctggggaatggagagggtaggggactaagtggcagggccgtgtcaagacccaggtctttcccaatgaacaaactcccctttacaaacagggagcaccccaaaaaataggaaggagctccacctgccccatcgtgacagtaactgacgtgttcctcaagggttatccaggcagtggaaccactcactgcagcagcatctccgagggtgggggcctgcacctggtgatcctgaggcacaccgcaggtgatggaacagtaccttcgtcctgcaggccactggtggcccaagacacacagctacagggctgggactgaggcgcccagtcttcatggtatcaacagcaggcttgaaggaatatactttattaatctacctcccaaacgctaaaatgccaaagactaaaatgctaacattcagctaaattaaaacaactatttacagagcactgtctgcaggccatgtggggctgggcccatttcttccccacccacccacccagcccatcctccaaacaggcctggggccacctgccacctgcagcagaaacacccagcacagaggacgtttatatacacctggccaagccctccacaatggcatgccaagaaggagggcaacagaccaagacagagaccgacagacagacagatagacatggacaggaggcgaggctgccaagaaggccgcaggccagcctcagtgcttcttcaggctgtaggccaggctgctggggaccctggcgccctgcaggggcggtgagttccagacagcagagctggtgcgcttgtgatagcggggcttgctcttcttgaagatatcctccaagtccagtgggagaatggttccaaagagctccagaaggttcggtgggtggtagtactggtgaatgatagcctggctgagcggggtgcctcgggcccaggtggggatgggcttccggggatgggcctcatcatcggtggagtcgtcgctattcagatccatcccgtagttatctgggttgatcttgggaggggccctgtgcccttgcggagtcatctgatatgaggtacaagctggagactgagagcctctccactggggcccaggtggcacctgcacgtccacagtcacattcagggccttgctggcccctgctgcctccttggctttcttctcttgctcctcctgcagctgccgctcagccagacgctgctgctcttccttcttcttcttctcctccagttccctctgcagctgctccttctgcagccgcagggccttctcccgctcctgcagctccctctcggcctggagccgctcctgctcccgccgacgctcctgctctgccagctgtcgctcctgctcgcgccgctcctgctcccgccgctcctgctcgcgccgctcctgctcgcgccgctcctgctcccgccgctcctgctcccgctgctctgccagccgcttagcctcggccgccttccgcagccgctcctgctcctcttccttcttcttctgcagcagctcttggtgccgccgctcttcctcctcctgctgcagccacctgagcctacgtgcctcctcttcctgcttcctgcgtgcttccacctcctccatcttcttggccgccgcctttttcttggccttctcctctgccagccgctcctccttggccttctcagtcttctcgtcgatctgagcaaacttctgctcaatctgcttcttcttctcctccttcatctgctccacccgctcgcgggcctgcagcaccttgcggaggcgttcctcacgcttcagcttcacctcctccagccgccgccgcttgtcctcctccaccttctgcctgcgcagctgctcggcctcctccttccgccgcagattctccaggcgctgccgctccttctccttggggtccatgcgcaggggagtgttgcgcttaataaaggacttcatgacgctgcgtggggctgaggtcggggtcatgagcatctggttcctctgcactgtgtgcagaaaggtccggaggggccgtaccaccttgctggctgggcagggtgaggaaggggtcttgctcctggggggctgcagctcctcatcctccaggtgctgctcctcgtccagctcactcacggcctgcttgtagctgcgcttcctcctggcactctgcggtggctctctgggtccatctgcttggtccgtcttggcctcttgctgccctgcagagggtgtttccgggctgctggctgcaggcttcgggttgggtgtgctgttggcaatctccgtgtcattgtggggccacgagttatttccattgttctcagggacctctggctcagctgccgccacaggctcagcctcctcggggggttccttctgctcagaaccaactttctggggcacctcaacattcaggagcctctccaggtaactgtgacagatgatgcggccagaggcagctggctcttcggcagtcttcttggcaagccttctgctcgccctgcggacaacactttcctgtttggccaccagagagtacttctgggctaagacttggggactcggggaagacggggcgatcgggctgtgccgcaccgattgagagtccgtgcgagagcccgtgggcgtggagaagttatccggcaggatgggagccagcacccgctcccgccatggagaatctggaaaggctggcgagtcccgtgggccaggggagacctgcgcaatcctgagcttagacgcagaccgccccgtcccgaccccttgacccttggggtcctggggtgtagccatcagggagctcactgtgatggactccagtatcctggccttcgacttcttaggtgttgattcctcatctgatgtcgggatgccctgggaggttggagctgtggctgaagctggagtcggggacagagtgcggggcagaggctcggtggacatgagctgggtgacatgctgctcagcattctggcgctcactgatgccgatctccaccacaggcaccagctggcactgggtgtggttatcctcgggcttcttagtcagcatcgtgggagactcaggggtgggtgaagaaggtgcagccaatgccatggtagccgcggcagctgcagccgcagcacgggtcacacgccgcaggacggagccgttctccccgaccactgtagccagcttctctacactgtccttgctgcggaggcgtcgggagctcagctggctgctccgagactttctgcgggataaccttctcctgatgggatctctgttttcatcctgaacataagaaatccgtctcttcttccgtcggttcttctgagaaggtgttttgggcatcagctctggctctttgctgaattctctggtgaacatgcgctcggcctcctcttggatttcctcaagccacaccaagtccttattatccatgttgcagagaaactccatgagcttctggtcacatagctccagcaggtgaatgggccctggggccgtcgtccccatggtggctctgttcgactgcgccacgtcccctgaaggctgctccgatccaagtccggtggtatccctaggtaaggccccgcttgcccagacccacttggctccgggccttcgggactcaccgcacgggaggagcaaccaggcggcgcagcgcgggcgaaaactatgattt

SEQ ID NO: 16519 - RNA, 3671 nt, Homo sapiens
  source 1..3671: mol_type = other RNA
gtggagtcctggggaatggagagggtaggggactaagtggcagggccgtgtcaagacccaggtctttcccaatgaacaaactcccctttacaaacagggagcaccccaaaaaataggaaggagctccacctgccccatcgtgacagtaactgacgtgttcctcaagggttatccaggcagtggaaccactcactgcagcagcatctccgagggtgggggcctgcacctggtgatcctgaggcacaccgcaggtgatggaacagtaccttcgtcctgcaggccactggtggcccaagacacacagctacagggctgggactgaggcgcccagtcttcatggtatcaacagcaggcttgaaggaatatactttattaatctacctcccaaacgctaaaatgccaaagactaaaatgctaacattcagctaaattaaaacaactatttacagagcactgtctgcaggccatgtggggctgggcccatttcttccccacccacccacccagcccatcctccaaacaggcctggggccacctgccacctgcagcagaaacacccagcacagaggacgtttatatacacctggccaagccctccacaatggcatgccaagaaggagggcaacagaccaagacagagaccgacagacagacagatagacatggacaggaggcgaggctgccaagaaggccgcaggccagcctcagtgcttcttcaggctgtaggccaggctgctggggaccctggcgccctgcaggggcggtgagttccagacagcagagctggtgcgcttgtgatagcggggcttgctcttcttgaagatatcctccaagtccagtgggagaatggttccaaagagctccagaaggttcggtgggtggtagtactggtgaatgatagcctggctgagcggggtgcctcgggcccaggtggggatgggcttccggggatgggcctcatcatcggtggagtcgtcgctattcagatccatcccgtagttatctgggttgatcttgggaggggccctgtgcccttgcggagtcatctgatatgaggtacaagctggagactgagagcctctccactggggcccaggtggcacctgcacgtccacagtcacattcagggccttgctggcccctgctgcctccttggctttcttctcttgctcctcctgcagctgccgctcagccagacgctgctgctcttccttcttcttcttctcctccagttccctctgcagctgctccttctgcagccgcagggccttctcccgctcctgcagctccctctcggcctggagccgctcctgctcccgccgacgctcctgctctgccagctgtcgctcctgctcgcgccgctcctgctcccgccgctcctgctcgcgccgctcctgctcgcgccgctcctgctcccgccgctcctgctcccgctgctctgccagccgcttagcctcggccgccttccgcagccgctcctgctcctcttccttcttcttctgcagcagctcttggtgccgccgctcttcctcctcctgctgcagccacctgagcctacgtgcctcctcttcctgcttcctgcgtgcttccacctcctccatcttcttggccgccgcctttttcttggccttctcctctgccagccgctcctccttggccttctcagtcttctcgtcgatctgagcaaacttctgctcaatctgcttcttcttctcctccttcatctgctccacccgctcgcgggcctgcagcaccttgcggaggcgttcctcacgcttcagcttcacctcctccagccgccgccgcttgtcctcctccaccttctgcctgcgcagctgctcggcctcctccttccgccgcagattctccaggcgctgccgctccttctcgacgaagctgcacttggggtccatgcgcaggggagtgttgcgcttaataaaggacttcatgacgctgcgtggggctgaggtcggggtcatgagcatctggttcctctgcactgtgtgcagaaaggtccggaggggccgtaccaccttgctggctgggcagggtgaggaaggggtcttgctcctggggggctgcagctcctcatcctccaggtgctgctcctcgtccagctcactcacggcctgcttgtagctgcgcttcctcctggcactctgcggtggctctctgggtccatctgcttggtccgtcttggcctcttgctgccctgcagagggtgtttccgggctgctggctgcaggcttcgggttgggtgtgctgttggcaatctccgtgtcattgtggggccacgagttatttccattgttctcagggacctctggctcagctgccgccacaggctcagcctcctcggggggttccttctgctcagaaccaactttctggggcacctcaacattcaggagcctctccaggtaactgtgacagatgatgcggccagaggcagctggctcttcggcagtcttcttggcaagccttctgctcgccctgcggacaacactttcctgtttggccaccagagagtacttctgggctaagacttggggactcggggaagacggggcgatcgggctgtgccgcaccgattgagagtccgtgcgagagcccgtgggcgtggagaagttatccggcaggatgggagccagcacccgctcccgccatggagaatctggaaaggctggcgagtcccgtgggccaggggagacctgcgcaatcctgagcttagacgcagaccgccccgtcccgaccccttgacccttggggtcctggggtgtagccatcagggagctcactgtgatggactccagtatcctggccttcgacttcttaggtgttgattcctcatctgatgtcgggatgccctgggaggttggagctgtggctgaagctggagtcggggacagagtgcggggcagaggctcggtggacatgagctgggtgacatgctgctcagcattctggcgctcactgatgccgatctccaccacaggcaccagctggcactgggtgtggttatcctcgggcttcttagtcagcatcgtgggagactcaggggtgggtgaagaaggtgcagccaatgccatggtagccgcggcagctgcagccgcagcacgggtcacacgccgcaggacggagccgttctccccgaccactgtagccagcttctctacactgtccttgctgcggaggcgtcgggagctcagctggctgctccgagactttctgcgggataaccttctcctgatgggatctctgttttcatcctgaacataagaaatccgtctcttcttccgtcggttcttctgagaaggtgttttgggcatcagctctggctctttgctgaattctctggtgaacatgcgctcggcctcctcttggatttcctcaagccacaccaagtccttattatccatgttgcagagaaactccatgagcttctggtcacatagctccagcaggtgaatgggccctggggccgtcgtccccatggtggctctgttcgactgcgccacgtcccctgaaggctgctccgatccaagtccggtggtatccctaggtaaggccccgcttgcccagacccacttggctccgggccttcgggactcaccgcacgggaggagcaaccaggcggcgcagcgcgggcgaaaactatgattttcaaaact

SEQ ID NO: 16520 - RNA, 3618 nt, Homo sapiens
  source 1..3618: mol_type = other RNA
gtggagtcctggggaatggagagggtaggggactaagtggcagggccgtgtcaagacccaggtctttcccaatgaacaaactcccctttacaaacagggagcaccccaaaaaataggaaggagctccacctgccccatcgtgacagtaactgacgtgttcctcaagggttatccaggcagtggaaccactcactgcagcagcatctccgagggtgggggcctgcacctggtgatcctgaggcacaccgcaggtgatggaacagtaccttcgtcctgcaggccactggtggcccaagacacacagctacagggctgggactgaggcgcccagtcttcatggtatcaacagcaggcttgaaggaatatactttattaatctacctcccaaacgctaaaatgccaaagactaaaatgctaacattcagctaaattaaaacaactatttacagagcactgtctgcaggccatgtggggctgggcccatttcttccccacccacccacccagcccatcctccaaacaggcctggggccacctgccacctgcagcagaaacacccagcacagaggacgtttatatacacctggccaagccctccacaatggcatgccaagaaggagggcaacagaccaagacagagaccgacagacagacagatagacatggacaggaggcgaggctgccaagaaggccgcaggccagcctcagtgcttcttcaggctgtaggccaggctgctggggaccctggcgccctgcaggggcggtgagttccagacagcagagctggtgcgcttgtgatagcggggcttgctcttcttgaagatatcctccaagtccagtgggagaatggttccaaagagctccagaaggttcggtgggtggtagtactggtgaatgatagcctggctgagcggggtgcctcgggcccaggtggggatgggcttccggggatgggcctcatcatcggtggagtcgtcgctattcagatccatcccgtagttatctgggttgatcttgggaggggccctgtgcccttgcggagtcatctgatatgaggtacaagctggagactgagagcctctccactggggcccaggtggcacctgcacgtccacagtcacattcagggccttgctggcccctgctgcctccttggctttcttctcttgctcctcctgcagctgccgctcagccagacgctgctgctcttccttcttcttcttctcctccagttccctctgcagctgctccttctgcagccgcagggccttctcccgctcctgcagctccctctcggcctggagccgctcctgctcccgccgacgctcctgctctgccagctgtcgctcctgctcgcgccgctcctgctcccgccgctcctgctcgcgccgctcctgctcgcgccgctcctgctcccgccgctcctgctcccgctgctctgccagccgcttagcctcggccgccttccgcagccgctcctgctcctcttccttcttcttctgcagcagctcttggtgccgccgctcttcctcctcctgtgctcgcacctgctgcagccacctgagcctacgtgcctcctcttcctgcttcctgcgtgcttccacctcctccatcttcttggccgccgcctttttcttggccttctcctctgccagccgctcctccttggccttctcagtcttctcgtcgatctgagcaaacttctgctcaatctgcttcttcttctcctccttcatctgctccacccgctcgcgggcctgcagcaccttgcggaggcgttcctcacgcttcagcttcacctcctccagccgccgccgcttgtcctcctccaccttctgcctgcgcagctgctcggcctcctccttccgccgcagattctccaggcgctgccgctccttctccttggggtccatgcgcaggggagtgttgcgcttaataaaggacttcatgacgctgcgtggggctgaggtcggggtcatgagcatctggttcctctgcactgtgtgcagaaaggtccggaggggccgtaccaccttgctggctgggcagggtgaggaaggggtcttgctcctggggggctgcagctcctcatcctccaggtgctgctcctcgtccagctcactcacggcctgcttgtagctgcgcttcctcctggcactctgcggtggctctctgggtccatctgcttggtccgtcttggcctcttgctgccctgcagagggtgtttccgggctgctggctgcaggcttcgggttgggtgtgctgttggcaatctccgtgtcattgtggggccacgagttatttccattgttctcagggacctctggctcagctgccgccacaggctcagcctcctcggggggttccttctgctcagaaccaactttctggggcacctcaacattcaggagcctctccaggtaactgtgacagatgatgcggccagaggcagctggctcttcggcagtcttcttggcaagccttctgctcgccctgcggacaacactttcctgtttggccaccagagagtacttctgggctaagacttggggactcggggaagacggggcgatcgggctgtgccgcaccgattgagagtccgtgcgagagcccgtgggcgtggagaagttatccggcaggatgggagccagcacccgctcccgccatggagaatctggaaaggctggcgagtcccgtgggccaggggagacctgcgcaatcctgagcttagacgcagaccgccccgtcccgaccccttgacccttggggtcctggggtgtagccatcagggagctcactgtgatggactccagtatcctggccttcgacttcttaggtgttgattcctcatctgatgtcgggatgccctgggaggttggagctgtggctgaagctggagtcggggacagagtgcggggcagaggctcggtggacatgagctgggtgacatgctgctcagcattctggcgctcactgatgccgatctccaccacaggcaccagctggcactgggtgtggttatcctcgggcttcttagtcagcatcgtgggagactcaggggtgggtgaagaaggtgcagccaatgccatggtagccgcggcagctgcagccgcagcacgggtcacacgccgcaggacggagccgttctccccgaccactgtagccagcttctctacactgtccttgctgcggaggcgtcgggagctcagctggctgctccgagactttctgcgggataaccttctcctgatgggatctctgttttcatcctgaacataagaaatccgtctcttcttccgtcggttcttctgagaaggtgttttgggcatcagctctggctctttgctgaattctctggtgaacatgcgctcggcctcctcttggatttcctcaagccacaccaagtccttattatccatgttgcagagaaactccatgagcttctggtcacatagctccagcaggtgaatgggccctggggccgtcgtccccatggtggctctgttcgactgcgccacgtcccctgaaggctgctccgatccaagtccggtggtatccctaggtaaggccccgcttgcccagacccacttggctccgggccttcgggactcaccgcac

SEQ ID NO: 16521 - RNA, 3683 nt, Homo sapiens
  source 1..3683: mol_type = other RNA
gtggagtcctggggaatggagagggtaggggactaagtggcagggccgtgtcaagacccaggtctttcccaatgaacaaactcccctttacaaacagggagcaccccaaaaaataggaaggagctccacctgccccatcgtgacagtaactgacgtgttcctcaagggttatccaggcagtggaaccactcactgcagcagcatctccgagggtgggggcctgcacctggtgatcctgaggcacaccgcaggtgatggaacagtaccttcgtcctgcaggccactggtggcccaagacacacagctacagggctgggactgaggcgcccagtcttcatggtatcaacagcaggcttgaaggaatatactttattaatctacctcccaaacgctaaaatgccaaagactaaaatgctaacattcagctaaattaaaacaactatttacagagcactgtctgcaggccatgtggggctgggcccatttcttccccacccacccacccagcccatcctccaaacaggcctggggccacctgccacctgcagcagaaacacccagcacagaggacgtttatatacacctggccaagccctccacaatggcatgccaagaaggagggcaacagaccaagacagagaccgacagacagacagatagacatggacaggaggcgaggctgccaagaaggccgcaggccagcctcagtgcttcttcaggctgtaggccaggctgctggggaccctggcgccctgcaggggcggtgagttccagacagcagagctggtgcgcttgtgatagcggggcttgctcttcttgaagatatcctccaagtccagtgggagaatggttccaaagagctccagaaggttcggtgggtggtagtactggtgaatgatagcctggctgagcggggtgcctcgggcccaggtggggatgggcttccggggatgggcctcatcatcggtggagtcgtcgctattcagatccatcccgtagttatctgggttgatcttgggaggggccctgtgcccttgcggagtcatctgatatgaggtacaagctggagactgagagcctctccactggggcccaggtggcacctgcacgtccacagtcacattcagggccttgctggcccctgctgcctccttggctttcttctcttgctcctcctgcagctgccgctcagccagacgctgctgctcttccttcttcttcttctcctccagttccctctgcagctgctccttctgcagccgcagggccttctcccgctcctgcagctccctctcggcctggagccgctcctgctcccgccgacgctcctgctctgccagctgtcgctcctgctcgcgccgctcctgctcccgccgctcctgctcgcgccgctcctgctcgcgccgctcctgctcccgccgctcctgctcccgctgctctgccagccgcttagcctcggccgccttccgcagccgctcctgctcctcttccttcttcttctgcagcagctcttggtgccgccgctcttcctcctcctgtgctcgcacctgctgcagccacctgagcctacgtgcctcctcttcctgcttcctgcgtgcttccacctcctccatcttcttggccgccgcctttttcttggccttctcctctgccagccgctcctccttggccttctcagtcttctcgtcgatctgagcaaacttctgctcaatctgcttcttcttctcctccttcatctgctccacccgctcgcgggcctgcagcaccttgcggaggcgttcctcacgcttcagcttcacctcctccagccgccgccgcttgtcctcctccaccttctgcctgcgcagctgctcggcctcctccttccgccgcagattctccaggcgctgccgctccttctcgacgaagctgcacttggggtccatgcgcaggggagtgttgcgcttaataaaggacttcatgacgctgcgtggggctgaggtcggggtcatgagcatctggttcctctgcactgtgtgcagaaaggtccggaggggccgtaccaccttgctggctgggcagggtgaggaaggggtcttgctcctggggggctgcagctcctcatcctccaggtgctgctcctcgtccagctcactcacggcctgcttgtagctgcgcttcctcctggcactctgcggtggctctctgggtccatctgcttggtccgtcttggcctcttgctgccctgcagagggtgtttccgggctgctggctgcaggcttcgggttgggtgtgctgttggcaatctccgtgtcattgtggggccacgagttatttccattgttctcagggacctctggctcagctgccgccacaggctcagcctcctcggggggttccttctgctcagaaccaactttctggggcacctcaacattcaggagcctctccaggtaactgtgacagatgatgcggccagaggcagctggctcttcggcagtcttcttggcaagccttctgctcgccctgcggacaacactttcctgtttggccaccagagagtacttctgggctaagacttggggactcggggaagacggggcgatcgggctgtgccgcaccgattgagagtccgtgcgagagcccgtgggcgtggagaagttatccggcaggatgggagccagcacccgctcccgccatggagaatctggaaaggctggcgagtcccgtgggccaggggagacctgcgcaatcctgagcttagacgcagaccgccccgtcccgaccccttgacccttggggtcctggggtgtagccatcagggagctcactgtgatggactccagtatcctggccttcgacttcttaggtgttgattcctcatctgatgtcgggatgccctgggaggttggagctgtggctgaagctggagtcggggacagagtgcggggcagaggctcggtggacatgagctgggtgacatgctgctcagcattctggcgctcactgatgccgatctccaccacaggcaccagctggcactgggtgtggttatcctcgggcttcttagtcagcatcgtgggagactcaggggtgggtgaagaaggtgcagccaatgccatggtagccgcggcagctgcagccgcagcacgggtcacacgccgcaggacggagccgttctccccgaccactgtagccagcttctctacactgtccttgctgcggaggcgtcgggagctcagctggctgctccgagactttctgcgggataaccttctcctgatgggatctctgttttcatcctgaacataagaaatccgtctcttcttccgtcggttcttctgagaaggtgttttgggcatcagctctggctctttgctgaattctctggtgaacatgcgctcggcctcctcttggatttcctcaagccacaccaagtccttattatccatgttgcagagaaactccatgagcttctggtcacatagctccagcaggtgaatgggccctggggccgtcgtccccatggtggctctgttcgactgcgccacgtcccctgaaggctgctccgatccaagtccggtggtatccctaggtaaggccccgcttgcccagacccacttggctccgggccttcgggactcaccgcacgggaggagcaaccaggcggcgcagcgcgggcgaaaactatgattttcaaaact

SEQ ID NO: 16522 - RNA, 3613 nt, Homo sapiens
  source 1..3613: mol_type = other RNA
gtggagtcctggggaatggagagggtaggggactaagtggcagggccgtgtcaagacccaggtctttcccaatgaacaaactcccctttacaaacagggagcaccccaaaaaataggaaggagctccacctgccccatcgtgacagtaactgacgtgttcctcaagggttatccaggcagtggaaccactcactgcagcagcatctccgagggtgggggcctgcacctggtgatcctgaggcacaccgcaggtgatggaacagtaccttcgtcctgcaggccactggtggcccaagacacacagctacagggctgggactgaggcgcccagtcttcatggtatcaacagcaggcttgaaggaatatactttattaatctacctcccaaacgctaaaatgccaaagactaaaatgctaacattcagctaaattaaaacaactatttacagagcactgtctgcaggccatgtggggctgggcccatttcttccccacccacccacccagcccatcctccaaacaggcctggggccacctgccacctgcagcagaaacacccagcacagaggacgtttatatacacctggccaagccctccacaatggcatgccaagaaggagggcaacagaccaagacagagaccgacagacagacagatagacatggacaggaggcgaggctgccaagaaggccgcaggccagcctcagtgcttcttcaggctgtaggccaggctgctggggaccctggcgccctgcaggggcggtgagttccagacagcagagctggtgcgcttgtgatagcggggcttgctcttcttgaagatatcctccaagtccagtgggagaatggttccaaagagctccagaaggttcggtgggtggtagtactggtgaatgatagcctggctgagcggggtgcctcgggcccaggtggggatgggcttccggggatgggcctcatcatcggtggagtcgtcgctattcagatccatcccgtagttatctgggttgatcttgggaggggccctgtgcccttgcggagtcatctgatatgaggtacaagctggagactgcacgtccacagtcacattcagggccttgctggcccctgctgcctccttggctttcttctcttgctcctcctgcagctgccgctcagccagacgctgctgctcttccttcttcttcttctcctccagttccctctgcagctgctccttctgcagccgcagggccttctcccgctcctgcagctccctctcggcctggagccgctcctgctcccgccgacgctcctgctctgccagctgtcgctcctgctcgcgccgctcctgctcccgccgctcctgctcgcgccgctcctgctcgcgccgctcctgctcccgccgctcctgctcccgctgctctgccagccgcttagcctcggccgccttccgcagccgctcctgctcctcttccttcttcttctgcagcagctcttggtgccgccgctcttcctcctcctgctgcagccacctgagcctacgtgcctcctcttcctgcttcctgcgtgcttccacctcctccatcttcttggccgccgcctttttcttggccttctcctctgccagccgctcctccttggccttctcagtcttctcgtcgatctgagcaaacttctgctcaatctgcttcttcttctcctccttcatctgctccacccgctcgcgggcctgcagcaccttgcggaggcgttcctcacgcttcagcttcacctcctccagccgccgccgcttgtcctcctccaccttctgcctgcgcagctgctcggcctcctccttccgccgcagattctccaggcgctgccgctccttctccttggggtccatgcgcaggggagtgttgcgcttaataaaggacttcatgacgctgcgtggggctgaggtcggggtcatgagcatctggttcctctgcactgtgtgcagaaaggtccggaggggccgtaccaccttgctggctgggcagggtgaggaaggggtcttgctcctggggggctgcagctcctcatcctccaggtgctgctcctcgtccagctcactcacggcctgcttgtagctgcgcttcctcctggcactctgcggtggctctctgggtccatctgcttggtccgtcttggcctcttgctgccctgcagagggtgtttccgggctgctggctgcaggcttcgggttgggtgtgctgttggcaatctccgtgtcattgtggggccacgagttatttccattgttctcagggacctctggctcagctgccgccacaggctcagcctcctcggggggttccttctgctcagaaccaactttctggggcacctcaacattcaggagcctctccaggtaactgtgacagatgatgcggccagaggcagctggctcttcggcagtcttcttggcaagccttctgctcgccctgcggacaacactttcctgtttggccaccagagagtacttctgggctaagacttggggactcggggaagacggggcgatcgggctgtgccgcaccgattgagagtccgtgcgagagcccgtgggcgtggagaagttatccggcaggatgggagccagcacccgctcccgccatggagaatctggaaaggctggcgagtcccgtgggccaggggagacctgcgcaatcctgagcttagacgcagaccgccccgtcccgaccccttgacccttggggtcctggggtgtagccatcagggagctcactgtgatggactccagtatcctggccttcgacttcttaggtgttgattcctcatctgatgtcgggatgccctgggaggttggagctgtggctgaagctggagtcggggacagagtgcggggcagaggctcggtggacatgagctgggtgacatgctgctcagcattctggcgctcactgatgccgatctccaccacaggcaccagctggcactgggtgtggttatcctcgggcttcttagtcagcatcgtgggagactcaggggtgggtgaagaaggtgcagccaatgccatggtagccgcggcagctgcagccgcagcacgggtcacacgccgcaggacggagccgttctccccgaccactgtagccagcttctctacactgtccttgctgcggaggcgtcgggagctcagctggctgctccgagactttctgcgggataaccttctcctgatgggatctctgttttcatcctgaacataagaaatccgtctcttcttccgtcggttcttctgagaaggtgttttgggcatcagctctggctctttgctgaattctctggtgaacatgcgctcggcctcctcttggatttcctcaagccacaccaagtccttattatccatgttgcagagaaactccatgagcttctggtcacatagctccagcaggtgaatgggccctggggccgtcgtccccatggtggctctgttcgactgcgccacgtcccctgaaggctgctccgatccaagtccggtggtatccctaggtaaggccccgcttgcccagacccacttggctccgggccttcgggactcaccgcacgggaggagcaaccaggcggcgcagcgcgggcgaaaactat

SEQ ID NO: 16523 - RNA, 3625 nt, Homo sapiens
  source 1..3625: mol_type = other RNA
gtggagtcctggggaatggagagggtaggggactaagtggcagggccgtgtcaagacccaggtctttcccaatgaacaaactcccctttacaaacagggagcaccccaaaaaataggaaggagctccacctgccccatcgtgacagtaactgacgtgttcctcaagggttatccaggcagtggaaccactcactgcagcagcatctccgagggtgggggcctgcacctggtgatcctgaggcacaccgcaggtgatggaacagtaccttcgtcctgcaggccactggtggcccaagacacacagctacagggctgggactgaggcgcccagtcttcatggtatcaacagcaggcttgaaggaatatactttattaatctacctcccaaacgctaaaatgccaaagactaaaatgctaacattcagctaaattaaaacaactatttacagagcactgtctgcaggccatgtggggctgggcccatttcttccccacccacccacccagcccatcctccaaacaggcctggggccacctgccacctgcagcagaaacacccagcacagaggacgtttatatacacctggccaagccctccacaatggcatgccaagaaggagggcaacagaccaagacagagaccgacagacagacagatagacatggacaggaggcgaggctgccaagaaggccgcaggccagcctcagtgcttcttcaggctgtaggccaggctgctggggaccctggcgccctgcaggggcggtgagttccagacagcagagctggtgcgcttgtgatagcggggcttgctcttcttgaagatatcctccaagtccagtgggagaatggttccaaagagctccagaaggttcggtgggtggtagtactggtgaatgatagcctggctgagcggggtgcctcgggcccaggtggggatgggcttccggggatgggcctcatcatcggtggagtcgtcgctattcagatccatcccgtagttatctgggttgatcttgggaggggccctgtgcccttgcggagtcatctgatatgaggtacaagctggagactgcacgtccacagtcacattcagggccttgctggcccctgctgcctccttggctttcttctcttgctcctcctgcagctgccgctcagccagacgctgctgctcttccttcttcttcttctcctccagttccctctgcagctgctccttctgcagccgcagggccttctcccgctcctgcagctccctctcggcctggagccgctcctgctcccgccgacgctcctgctctgccagctgtcgctcctgctcgcgccgctcctgctcccgccgctcctgctcgcgccgctcctgctcgcgccgctcctgctcccgccgctcctgctcccgctgctctgccagccgcttagcctcggccgccttccgcagccgctcctgctcctcttccttcttcttctgcagcagctcttggtgccgccgctcttcctcctcctgctgcagccacctgagcctacgtgcctcctcttcctgcttcctgcgtgcttccacctcctccatcttcttggccgccgcctttttcttggccttctcctctgccagccgctcctccttggccttctcagtcttctcgtcgatctgagcaaacttctgctcaatctgcttcttcttctcctccttcatctgctccacccgctcgcgggcctgcagcaccttgcggaggcgttcctcacgcttcagcttcacctcctccagccgccgccgcttgtcctcctccaccttctgcctgcgcagctgctcggcctcctccttccgccgcagattctccaggcgctgccgctccttctcgacgaagctgcacttggggtccatgcgcaggggagtgttgcgcttaataaaggacttcatgacgctgcgtggggctgaggtcggggtcatgagcatctggttcctctgcactgtgtgcagaaaggtccggaggggccgtaccaccttgctggctgggcagggtgaggaaggggtcttgctcctggggggctgcagctcctcatcctccaggtgctgctcctcgtccagctcactcacggcctgcttgtagctgcgcttcctcctggcactctgcggtggctctctgggtccatctgcttggtccgtcttggcctcttgctgccctgcagagggtgtttccgggctgctggctgcaggcttcgggttgggtgtgctgttggcaatctccgtgtcattgtggggccacgagttatttccattgttctcagggacctctggctcagctgccgccacaggctcagcctcctcggggggttccttctgctcagaaccaactttctggggcacctcaacattcaggagcctctccaggtaactgtgacagatgatgcggccagaggcagctggctcttcggcagtcttcttggcaagccttctgctcgccctgcggacaacactttcctgtttggccaccagagagtacttctgggctaagacttggggactcggggaagacggggcgatcgggctgtgccgcaccgattgagagtccgtgcgagagcccgtgggcgtggagaagttatccggcaggatgggagccagcacccgctcccgccatggagaatctggaaaggctggcgagtcccgtgggccaggggagacctgcgcaatcctgagcttagacgcagaccgccccgtcccgaccccttgacccttggggtcctggggtgtagccatcagggagctcactgtgatggactccagtatcctggccttcgacttcttaggtgttgattcctcatctgatgtcgggatgccctgggaggttggagctgtggctgaagctggagtcggggacagagtgcggggcagaggctcggtggacatgagctgggtgacatgctgctcagcattctggcgctcactgatgccgatctccaccacaggcaccagctggcactgggtgtggttatcctcgggcttcttagtcagcatcgtgggagactcaggggtgggtgaagaaggtgcagccaatgccatggtagccgcggcagctgcagccgcagcacgggtcacacgccgcaggacggagccgttctccccgaccactgtagccagcttctctacactgtccttgctgcggaggcgtcgggagctcagctggctgctccgagactttctgcgggataaccttctcctgatgggatctctgttttcatcctgaacataagaaatccgtctcttcttccgtcggttcttctgagaaggtgttttgggcatcagctctggctctttgctgaattctctggtgaacatgcgctcggcctcctcttggatttcctcaagccacaccaagtccttattatccatgttgcagagaaactccatgagcttctggtcacatagctccagcaggtgaatgggccctggggccgtcgtccccatggtggctctgttcgactgcgccacgtcccctgaaggctgctccgatccaagtccggtggtatccctaggtaaggccccgcttgcccagacccacttggctccgggccttcgggactcaccgcacgggaggagcaaccaggcggcgcagcgcgggcgaaaactat

SEQ ID NO: 16524 - RNA, 3650 nt, Homo sapiens
  source 1..3650: mol_type = other RNA
gtggagtcctggggaatggagagggtaggggactaagtggcagggccgtgtcaagacccaggtctttcccaatgaacaaactcccctttacaaacagggagcaccccaaaaaataggaaggagctccacctgccccatcgtgacagtaactgacgtgttcctcaagggttatccaggcagtggaaccactcactgcagcagcatctccgagggtgggggcctgcacctggtgatcctgaggcacaccgcaggtgatggaacagtaccttcgtcctgcaggccactggtggcccaagacacacagctacagggctgggactgaggcgcccagtcttcatggtatcaacagcaggcttgaaggaatatactttattaatctacctcccaaacgctaaaatgccaaagactaaaatgctaacattcagctaaattaaaacaactatttacagagcactgtctgcaggccatgtggggctgggcccatttcttccccacccacccacccagcccatcctccaaacaggcctggggccacctgccacctgcagcagaaacacccagcacagaggacgtttatatacacctggccaagccctccacaatggcatgccaagaaggagggcaacagaccaagacagagaccgacagacagacagatagacatggacaggaggcgaggctgccaagaaggccgcaggccagcctcagtgcttcttcaggctgtaggccaggctgctggggaccctggcgccctgcaggggcggtgagttccagacagcagagctggtgcgcttgtgatagcggggcttgctcttcttgaagatatcctccaagtccagtgggagaatggttccaaagagctccagaaggttcggtgggtggtagtactggtgaatgatagcctggctgagcggggtgcctcgggcccaggtggggatgggcttccggggatgggcctcatcatcggtggagtcgtcgctattcagatccatcccgtagttatctgggttgatcttgggaggggccctgtgcccttgcggagtcatctgatatgaggtacaagctggagactgcacgtccacagtcacattcagggccttgctggcccctgctgcctccttggctttcttctcttgctcctcctgcagctgccgctcagccagacgctgctgctcttccttcttcttcttctcctccagttccctctgcagctgctccttctgcagccgcagggccttctcccgctcctgcagctccctctcggcctggagccgctcctgctcccgccgacgctcctgctctgccagctgtcgctcctgctcgcgccgctcctgctcccgccgctcctgctcgcgccgctcctgctcgcgccgctcctgctcccgccgctcctgctcccgctgctctgccagccgcttagcctcggccgccttccgcagccgctcctgctcctcttccttcttcttctgcagcagctcttggtgccgccgctcttcctcctcctgtgctcgcacctgctgcagccacctgagcctacgtgcctcctcttcctgcttcctgcgtgcttccacctcctccatcttcttggccgccgcctttttcttggccttctcctctgccagccgctcctccttggccttctcagtcttctcgtcgatctgagcaaacttctgctcaatctgcttcttcttctcctccttcatctgctccacccgctcgcgggcctgcagcaccttgcggaggcgttcctcacgcttcagcttcacctcctccagccgccgccgcttgtcctcctccaccttctgcctgcgcagctgctcggcctcctccttccgccgcagattctccaggcgctgccgctccttctcgacgaagctgcacttggggtccatgcgcaggggagtgttgcgcttaataaaggacttcatgacgctgcgtggggctgaggtcggggtcatgagcatctggttcctctgcactgtgtgcagaaaggtccggaggggccgtaccaccttgctggctgggcagggtgaggaaggggtcttgctcctggggggctgcagctcctcatcctccaggtgctgctcctcgtccagctcactcacggcctgcttgtagctgcgcttcctcctggcactctgcggtggctctctgggtccatctgcttggtccgtcttggcctcttgctgccctgcagagggtgtttccgggctgctggctgcaggcttcgggttgggtgtgctgttggcaatctccgtgtcattgtggggccacgagttatttccattgttctcagggacctctggctcagctgccgccacaggctcagcctcctcggggggttccttctgctcagaaccaactttctggggcacctcaacattcaggagcctctccaggtaactgtgacagatgatgcggccagaggcagctggctcttcggcagtcttcttggcaagccttctgctcgccctgcggacaacactttcctgtttggccaccagagagtacttctgggctaagacttggggactcggggaagacggggcgatcgggctgtgccgcaccgattgagagtccgtgcgagagcccgtgggcgtggagaagttatccggcaggatgggagccagcacccgctcccgccatggagaatctggaaaggctggcgagtcccgtgggccaggggagacctgcgcaatcctgagcttagacgcagaccgccccgtcccgaccccttgacccttggggtcctggggtgtagccatcagggagctcactgtgatggactccagtatcctggccttcgacttcttaggtgttgattcctcatctgatgtcgggatgccctgggaggttggagctgtggctgaagctggagtcggggacagagtgcggggcagaggctcggtggacatgagctgggtgacatgctgctcagcattctggcgctcactgatgccgatctccaccacaggcaccagctggcactgggtgtggttatcctcgggcttcttagtcagcatcgtgggagactcaggggtgggtgaagaaggtgcagccaatgccatggtagccgcggcagctgcagccgcagcacgggtcacacgccgcaggacggagccgttctccccgaccactgtagccagcttctctacactgtccttgctgcggaggcgtcgggagctcagctggctgctccgagactttctgcgggataaccttctcctgatgggatctctgttttcatcctgaacataagaaatccgtctcttcttccgtcggttcttctgagaaggtgttttgggcatcagctctggctctttgctgaattctctggtgaacatgcgctcggcctcctcttggatttcctcaagccacaccaagtccttattatccatgttgcagagaaactccatgagcttctggtcacatagctccagcaggtgaatgggccctggggccgtcgtccccatggtggctctgttcgactgcgccacgtcccctgaaggctgctccgatccaagtccggtggtatccctaggtaaggccccgcttgcccagacccacttggctccgggccttcgggactcaccgcacgggaggagcaaccaggcggcgcagcgcgggcgaaaactatgattttcaaaact

SEQ ID NO: 16525 - RNA, 3746 nt, Homo sapiens
  source 1..3746: mol_type = other RNA
gtgggcgggggcaggtgtgtggctgacagtggggagcctgctggggacgccaagggtgctgtttcctgcttaatcagggacacctctgtccccttctagctttccagggataactgggatgctcccacgccccctgtgtggctcagggatgaggcacttctctctcagccactcaactgatggaaggaaaaggcgatggaaagtctaacttttctgaaacaggtaggtgacaccttttggaaccggaatcaatcattattcttgcgtgggttttccattttccctgaagcatcgcaccagcttttgcgcgatgcctcggcttaccattttgcatctatcttaaggaattaggaggattcagaggagggtttctacgggcctctgctcacttttcacctctagggagactcaagtttccaagcattctttctgcaaagcacctgcctttgctaccttattgccgtattaccagccatcattttgattcatcttgaatactacagattaaaaaatattccctgcataatggctttgtgcaaaaacaagggaaagaaaacagaaagaagaaaggaaaatgtcctatcagaaagtggtcctccatgtttgcagaaaacccaggacccaccgggccctggtgggagcgggaagccgcctgccctgggagagggtgcccatcggtcaggatgcccggctggcctgcccagccccgctggcatagctacaggacgcccccgtggtaggcatggctgggggctgggctgccgaggctgtctgggcaggctttggtgttgtggtggttgcacggcggctcgtccttctgccgctccttctccatccaggtttccagcagctgctgcttgtcttgctcctcccgcatgaacagctccaccatgagcaccttctccttgtggatctgctggctgatgtccttggggatgtccgggatgacccagtccacaaagtcgctcatgaacatgaccaggttctggaagacgatgacaaacgccagccgggctgccaggacggcccagaagtccttggagatgtcgtacttgttttccgaccacggcggctctcggtagtctttatacctgcagatctgcacctcgtagcccaggtccagggggtcattgggggccgtgccgttctggaagtcactgacgttgaaggaggagagggtgtggttgacgaagccgtgcatggtcccgttcttactgtacatgtagaggtacaccaggcgcgggatgaagtcagacgtgaaggagatcacgaaggcattgatgatgacagcaagcttcccaatgcctctgaggatattgtaccagattccgatgtctttggctctgacagctaccggccttcggagctcagtgacaaactttttggcgtccaggcggatctcgatgatgttgttcagcagcgcaaacagtggggccagggggaaggaggcgacaaacagggtgacgaagccaaactggatgatcatttccatgtactctggggtgaggcccgcgaagggctccaggttgtaatccacctcgtaccgctgtttcctcttcacacactcctcgtggtcaggggggctctgctgcttcagcttcaggtagcggatgagcttcttcatcttcgggatgccgatctcgaacaggttgttctggatcagctgtttccccagcatgatgatgctgagctggatgcatagctccatcaggcagccccctggcgcacactcttccattcggaaggaacggaaaatgtacacgtagtcgcccgggcgtccaacaaaccggcctttgaagaacgccacgtaaaagatgggggtgtaggaattcacaaacttcagcaggaaagccttgaagatcagcctctcctcaaagcttttctccgtctttgggacctcgatcttggtgagccatcgggctatgcagccatacacctcgtccaggaggatgatgaccactaggttgatgatgactgcggtggctgtgactgtgacccggatgttggaccgcacggagggggaggagttcatggccaaggcggcggccatggagattctgtagatgatgacgccgaggacgatggcaaacgtcactgcaatcatgaagatgatggagaccaagttagtgaggtaggctgggaaccgatctctccatgtcagcttcactttgtcagtcaatttcacccccgccatggctgtcttaaccctctgcttccatttgtttgttgactcctctggaatatgccggcgcttctctttgtttctggactctttcttcagagacttctccaagactctggcttcgtattcagctctaggatgatcctcttcctcttcaaagcccgtgaggtcccagcggtagttgagtcgcatctgtttccgcttccagtgctccatgaaggtggcagcccagagggccatgaagacagagaagaagaccgtggcggggttgtcgaagaggtggctggcgcgggccgtggcgcaggctgagctcatcttccagtagctgcaggtcttgtcgcaaagcgggcacatggtgatattgtgtctctggtcacacatctccatgctggggatgttttcatccatggtggcgcatccgtacaggaagacaatgattcccacgatggaggcagggatgagcatctgggtgtacacgcccagccaggcgaagtacaggccgatcttctccccaaaatacttcctgaccaggtcgatgggctggtacttatagaaaactccatagcgtgcccactcttcgtacaggagttttctgtcgttgaactcgacgttttcaccgttgtagtctccatcgtgcagtgggtatgcagccgcgtacacaccattggccagcaggctcgtgatgccatacttcccacatttccgccttttacttagaagggcggagtccttctttcttccctcgccttgccccatgctgtacttggcctttgtacacgtcgttctcttcaagatctcatagacaatcgtgctccgggttttgctgtcgaaaaaggaatccttatcagacaagtcaaatagatgctgcttctcccgggagaagggataggagagtctcttcatggtctggggcctgtgctcagccactttgggctggatgggatctgtgattttctggagcacagagttgatttttttcaggaggccacgggtctcattaatgtggtacatcttcttcgtcggcatcttcagtttcagaaactcggcctctctgcacagcacgttccagggggcatggattttcacaaacccgactccgtggattttagtgtcctcgtcccgctccagctccaggcccgcctccaggaggttgccctcgtactcctccctgcggaagcgcttgtcatcctcgtggtagtccatcgggggctcccccgagcctgcatccagcgacgcccccttgcccggcagggggtggtcctgcttgacgctgcgagccccagagggggtgtcgctgtgctgcaccctcctgaccagggtccggttgcccgagggcctcttgtgatggtacaccaggatgtagtccaccttgcgccggccgtccctgaagtacaggccatacttgcactcggcatcagggtccacagataaggagttcagcagcgtgccctcggacggcaggtagccgatgtcctcgatggcgcagatgttgatgatgtggacgctgcggtcctcggccgggagcgtcgagtacttctcgttgaccctcatcgtggccgcctgt

SEQ ID NO: 16526 - RNA, 3734 nt, Homo sapiens
  source 1..3734: mol_type = other RNA
gtgggcgggggcaggtgtgtggctgacagtggggagcctgctggggacgccaagggtgctgtttcctgcttaatcagggacacctctgtccccttctagctttccagggataactgggatgctcccacgccccctgtgtggctcagggatgaggcacttctctctcagccactcaactgatggaaggaaaaggcgatggaaagtctaacttttctgaaacaggtaggtgacaccttttggaaccggaatcaatcattattcttgcgtgggttttccattttccctgaagcatcgcaccagcttttgcgcgatgcctcggcttaccattttgcatctatcttaaggaattaggaggattcagaggagggtttctacgggcctctgctcacttttcacctctagggagactcaagtttccaagcattctttctgcaaagcacctgcctttgctaccttattgccgtattaccagccatcattttgattcatcttgaatactacagattaaaaaatattccctgcataatggctttgtgcaaaaacaagggaaagaaaacagaaagaagaaaggaaaatgtcctatcagaaagtggtcctccatgtttgcagaaaacccaggacccaccgggccctggtgggagcgggaagccgcctgccctgggagagggtgcccatcggtcaggatgcccggctggcctgcccagccccgctggcatagctacaggacgcccccgtggtaggcatggctgggggctgggctgccgaggctgtctgggcaggctttggtgttgtggtggttgcacggcggctcgtccttctgccgctccttctccatccaggtttccagcagctgctgcttgtcttgctcctcccgcatgaacagctccaccatgagcaccttctccttgtggatctgctggctgatgtccttggggatgtccgggatgacccagtccacaaagtcgctcatgaacatgaccaggttctggaagacgatgacaaacgccagccgggctgccaggacggcccagaagtccttggagatgtcgtacttgttttccgaccacggcggctctcggtagtctttatacctgcagatctgcacctcgtagcccaggtccagggggtcattgggggccgtgccgttctggaagtcactgacgttgaaggaggagagggtgtggttgacgaagccgtgcatggtcccgttcttactgtacatgtagaggtacaccaggcgcgggatgaagtcagacgtgaaggagatcacgaaggcattgatgatgacagcaagcttcccaatgcctctgaggatattgtaccagattccgatgtctttggctctgacagctaccggccttcggagctcagtgacaaactttttggcgtccaggcggatctcgatgatgttgttcagcagcgcaaacagtggggccagggggaaggaggcgacaaacagggtgacgaagccaaactggatgatcatttccatgtactctggggtgaggcccgcgaagggctccaggttgtaatccacctcgtaccgctgtttcctcttcacacactcctcgtggtcaggggggctctgctgcttcagcttcaggtagcggatgagcttcttcatcttcgggatgccgatctcgaacaggttgttctggatcagctgtttccccagcatgatgatgctgagctggatgcatagctccatcaggcagccccctggcgcacactcttccattcggaaggaacggaaaatgtacacgtagtcgcccgggcgtccaacaaaccggcctttgaagaacgccacgtaaaagatgggggtgtaggaattcacaaacttcagcaggaaagccttgaagatcagcctctcctcaaagcttttctccgtctttgggacctcgatcttggtgagccatcgggctatgcagccatacacctcgtccaggaggatgatgaccactaggttgatgatgactgcggtggctgtgactgtgacccggatgttggaccgcacggagggggaggagttcatggccaaggcggcggccatggagattctgtagatgatgacgccgaggacgatggcaaacgtcactgcaatcatgaagatgatggagaccaagttagtgaggtaggctgggaaccgatctctccatgtcagcttcactttgtcagtcaatttcacccccgccatggctgtcttaaccctctgcttccatttgtttgttgactcctctggaatatgccggcgcttctctttgtttctggactctttcttcagagacttctccaagactctggcttcgtattcagctctaggatgatcctcttcctcttcaaagcccgtgaggtcccagcggtagttgagtcgcatctgtttccgcttccagtgctccatgaaggtggcagcccagagggccatgaagacagagaagaagaccgtggcggggttgtcgaagaggtggctggcgcgggccgtggcgcaggctgagctcatcttccagtagctgcaggtcttgtcgcaaagcgggcacatggtgatattgtgtctctggtcacacatctccatgctggggatgttttcatccatggtggcgcatccgtacaggaagacaatgattcccacgatggaggcagggatgagcatctgggtgtacacgcccagccaggcgaagtacaggccgatcttctccccaaaatacttcctgaccaggtcgatgggctggtacttatagaaaactccatagcgtgcccactcttcgtacaggagttttctgtcgttgaactcgacgttttcaccgttgtagtctccatcgtgcagtgggtatgcagccgcgtacacaccattggccagcaggctcgtgatgcccatgctgtacttggcctttgtacacgtcgttctcttcaagatctcatagacaatcgtgctccgggttttgctgtcgaaaaaggaatccttatcagacaagtcaaatagatgctgcttctcccgggagaagggataggagagtctcttcatggtctggggcctgtgctcagccactttgggctggatgggatctgtgattttctggagcacagagttgatttttttcaggaggccacgggtctcattaatgtggtacatcttcttcgtcggcatcttcagtttcagaaactcggcctctctgcacagcacgttccagggggcatggattttcacaaacccgactccgtggattttagtgtcctcgtcccgctccagctccaggcccgcctccaggaggttgccctcgtactcctccctgcggaagcgcttgtcatcctcgtggtagtccatcgggggctcccccgagcctgcatccagcgacgcccccttgcccggcagggggtggtcctgcttgacgctgcgagccccagagggggtgtcgctgtgctgcaccctcctgaccagggtccggttgcccgagggcctcttgtgatggtacaccaggatgtagtccaccttgcgccggccgtccctgaagtacaggccatacttgcactcggcatcagggtccacagataaggagttcagcagcgtgccctcggacggcaggtagccgatgtcctcgatggcgcagatgttgatgatgtggacgctgcggtcctcggccgggagcgtcgagtacttctcgttgaccctcatcgtggccgcctgtgcgctgggaccgccgggcggcgcgccctccccatccacggccccggcggcctct

SEQ ID NO: 16527 - RNA, 3805 nt, Homo sapiens
  source 1..3805: mol_type = other RNA
gtgggcgggggcaggtgtgtggctgacagtggggagcctgctggggacgccaagggtgctgtttcctgcttaatcagggacacctctgtccccttctagctttccagggataactgggatgctcccacgccccctgtgtggctcagggatgaggcacttctctctcagccactcaactgatggaaggaaaaggcgatggaaagtctaacttttctgaaacaggtaggtgacaccttttggaaccggaatcaatcattattcttgcgtgggttttccattttccctgaagcatcgcaccagcttttgcgcgatgcctcggcttaccattttgcatctatcttaaggaattaggaggattcagaggagggtttctacgggcctctgctcacttttcacctctagggagactcaagtttccaagcattctttctgcaaagcacctgcctttgctaccttattgccgtattaccagccatcattttgattcatcttgaatactacagattaaaaaatattccctgcataatggctttgtgcaaaaacaagggaaagaaaacagaaagaagaaaggaaaatgtcctatcagaaagtggtcctccatgtttgcagaaaacccaggacccaccgggccctggtgggagcgggaagccgcctgccctgggagagggtgcccatcggtcaggatgcccggctggcctgcccagccccgctggcatagctacaggacgcccccgtggtaggcatggctgggggctgggctgccgaggctgtctgggcaggctttggtgttgtggtggttgcacggcggctcgtccttctgccgctccttctccatccaggtttccagcagctgctgcttgtcttgctcctcccgcatgaacagctccaccatgagcaccttctccttgtggatctgctggctgatgtccttggggatgtccgggatgacccagtccacaaagtcgctcatgaacatgaccaggttctggaagacgatgacaaacgccagccgggctgccaggacggcccagaagtccttggagatgtcgtacttgttttccgaccacggcggctctcggtagtctttatacctgcagatctgcacctcgtagcccaggtccagggggtcattgggggccgtgccgttctggaagtcactgacgttgaaggaggagagggtgtggttgacgaagccgtgcatggtcccgttcttactgtacatgtagaggtacaccaggcgcgggatgaagtcagacgtgaaggagatcacgaaggcattgatgatgacagcaagcttcccaatgcctctgaggatattgtaccagattccgatgtctttggctctgacagctaccggccttcggagctcagtgacaaactttttggcgtccaggcggatctcgatgatgttgttcagcagcgcaaacagtggggccagggggaaggaggcgacaaacagggtgacgaagccaaactggatgatcatttccatgtactctggggtgaggcccgcgaagggctccaggttgtaatccacctcgtaccgctgtttcctcttcacacactcctcgtggtcaggggggctctgctgcttcagcttcaggtagcggatgagcttcttcatcttcgggatgccgatctcgaacaggttgttctggatcagctgtttccccagcatgatgatgctgagctggatgcatagctccatcaggcagccccctggcgcacactcttccattcggaaggaacggaaaatgtacacgtagtcgcccgggcgtccaacaaaccggcctttgaagaacgccacgtaaaagatgggggtgtaggaattcacaaacttcagcaggaaagccttgaagatcagcctctcctcaaagcttttctccgtctttgggacctcgatcttggtgagccatcgggctatgcagccatacacctcgtccaggaggatgatgaccactaggttgatgatgactgcggtggctgtgactgtgacccggatgttggaccgcacggagggggaggagttcatggccaaggcggcggccatggagattctgtagatgatgacgccgaggacgatggcaaacgtcactgcaatcatgaagatgatggagaccaagttagtgaggtaggctgggaaccgatctctccatgtcagcttcactttgtcagtcaatttcacccccgccatggctgtcttaaccctctgcttccatttgtttgttgactcctctggaatatgccggcgcttctctttgtttctggactctttcttcagagacttctccaagactctggcttcgtattcagctctaggatgatcctcttcctcttcaaagcccgtgaggtcccagcggtagttgagtcgcatctgtttccgcttccagtgctccatgaaggtggcagcccagagggccatgaagacagagaagaagaccgtggcggggttgtcgaagaggtggctggcgcgggccgtggcgcaggctgagctcatcttccagtagctgcaggtcttgtcgcaaagcgggcacatggtgatattgtgtctctggtcacacatctccatgctggggatgttttcatccatggtggcgcatccgtacaggaagacaatgattcccacgatggaggcagggatgagcatctgggtgtacacgcccagccaggcgaagtacaggccgatcttctccccaaaatacttcctgaccaggtcgatgggctggtacttatagaaaactccatagcgtgcccactcttcgtacaggagttttctgtcgttgaactcgacgttttcaccgttgtagtctccatcgtgcagtgggtatgcagccgcgtacacaccattggccagcaggctcgtgatgcccatgctgtacttggcctttgtacacgtcgttctcttcaagatctcatagacaatcgtgctccgggttttgctgtcgaaaaaggaatccttatcagacaagtcaaatagatgctgcttctcccgggagaagggataggagagtctcttcatggtctggggcctgtgctcagccactttgggctggatgggatctgtgattttctggagcacagagttgatttttttcaggaggccacgggtctcattaatgtggtacatcttcttcgtcggcatcttcagtttcagaaactcggcctctctgcacagcacgttccagggggcatggattttcacaaacccgactccgtggattttagtgtcctcgtcccgctccagctccaggcccgcctccaggaggttgccctcgtactcctccctgcggaagcgcttgtcatcctcgtggtagtccatcgggggctcccccgagcctgcatccagcgacgcccccttgcccggcagggggtggtcctgcttgacgctgcgagccccagagggggtgtcgctgtgctgcaccctcctgaccagggtccggttgcccgagggcctcttgtgatggtacaccaggatgtagtccaccttgcgccggccgtccctgaagtacaggccatacttgcactcggcatcagggtccacagataaggagttcagcagcgtgccctcggacggcaggtagccgatgtcctcgatggcgcagatgttgatgatgtggacgctgcggtcctcggccgggagcgtcgagtacttctcgttgaccctcatcgtggccgcctgtgcgctgggaccgccgggcggcgcgccctccccatccacggccccggcggcctctgaaataaagtccccgagtggcaggcgcttctgtggcgcgtcacctccgcctccggggggagtgaagcttct

SEQ ID NO: 16528 - RNA, 3766 nt, Homo sapiens
  source 1..3766: mol_type = other RNA
gtgggcgggggcaggtgtgtggctgacagtggggagcctgctggggacgccaagggtgctgtttcctgcttaatcagggacacctctgtccccttctagctttccagggataactgggatgctcccacgccccctgtgtggctcagggatgaggcacttctctctcagccactcaactgatggaaggaaaaggcgatggaaagtctaacttttctgaaacaggtaggtgacaccttttggaaccggaatcaatcattattcttgcgtgggttttccattttccctgaagcatcgcaccagcttttgcgcgatgcctcggcttaccattttgcatctatcttaaggaattaggaggattcagaggagggtttctacgggcctctgctcacttttcacctctagggagactcaagtttccaagcattctttctgcaaagcacctgcctttgctaccttattgccgtattaccagccatcattttgattcatcttgaatactacagattaaaaaatattccctgcataatggctttgtgcaaaaacaagggaaagaaaacagaaagaagaaaggaaaatgtcctatcagaaagtggtcctccatgtttgcagaaaacccaggacccaccgggccctggtgggagcgggaagccgcctgccctgggagagggtgcccatcggtcaggatgcccggctggcctgcccagccccgctggcatagctacaggacgcccccgtggtaggcatggctgggggctgggctgccgaggctgtctgggcaggctttggtgttgtggtggttgcacggcggctcgtccttctgccgctccttctccatccaggtttccagcagctgctgcttgtcttgctcctcccgcatgaacagctccaccatgagcaccttctccttgtggatctgctggctgatgtccttggggatgtccgggatgacccagtccacaaagtcgctcatgaacatgaccaggttctggaagacgatgacaaacgccagccgggctgccaggacggcccagaagtccttggagatgtcgtacttgttttccgaccacggcggctctcggtagtctttatacctgcagatctgcacctcgtagcccaggtccagggggtcattgggggccgtgccgttctggaagtcactgacgttgaaggaggagagggtgtggttgacgaagccgtgcatggtcccgttcttactgtacatgtagaggtacaccaggcgcgggatgaagtcagacgtgaaggagatcacgaaggcattgatgatgacagcaagcttcccaatgcctctgaggatattgtaccagattccgatgtctttggctctgacagctaccggccttcggagctcagtgacaaactttttggcgtccaggcggatctcgatgatgttgttcagcagcgcaaacagtggggccagggggaaggaggcgacaaacagggtgacgaagccaaactggatgatcatttccatgtactctggggtgaggcccgcgaagggctccaggttgtaatccacctcgtaccgctgtttcctcttcacacactcctcgtggtcaggggggctctgctgcttcagcttcaggtagcggatgagcttcttcatcttcgggatgccgatctcgaacaggttgttctggatcagctgtttccccagcatgatgatgctgagctggatgcatagctccatcaggcagccccctggcgcacactcttccattcggaaggaacggaaaatgtacacgtagtcgcccgggcgtccaacaaaccggcctttgaagaacgccacgtaaaagatgggggtgtaggaattcacaaacttcagcaggaaagccttgaagatcagcctctcctcaaagcttttctccgtctttgggacctcgatcttggtgagccatcgggctatgcagccatacacctcgtccaggaggatgatgaccactaggttgatgatgactgcggtggctgtgactgtgacccggatgttggaccgcacggagggggaggagttcatggccaaggcggcggccatggagattctgtagatgatgacgccgaggacgatggcaaacgtcactgcaatcatgaagatgatggagaccaagttagtgaggtaggctgggaaccgatctctccatgtcagcttcactttgtcagtcaatttcacccccgccatggctgtcttaaccctctgcttccatttgtttgttgactcctctggaatatgccggcgcttctctttgtttctggactctttcttcagagacttctccaagactctggcttcgtattcagctctaggatgatccttgacagcctcctcttcctcttcaaagcccgtgaggtcccagcggtagttgagtcgcatctgtttccgcttccagtgctccatgaaggtggcagcccagagggccatgaagacagagaagaagaccgtggcggggttgtcgaagaggtggctggcgcgggccgtggcgcaggctgagctcatcttccagtagctgcaggtcttgtcgcaaagcgggcacatggtgatattgtgtctctggtcacacatctccatgctggggatgttttcatccatggtggcgcatccgtacaggaagacaatgattcccacgatggaggcagggatgagcatctgggtgtacacgcccagccaggcgaagtacaggccgatcttctccccaaaatacttcctgaccaggtcgatgggctggtacttatagaaaactccatagcgtgcccactcttcgtacaggagttttctgtcgttgaactcgacgttttcaccgttgtagtctccatcgtgcagtgggtatgcagccgcgtacacaccattggccagcaggctcgtgatgccatacttcccacatttccgccttttacttagaagggcggagtccttctttcttccctcgccttgccccatgctgtacttggcctttgtacacgtcgttctcttcaagatctcatagacaatcgtgctccgggttttgctgtcgaaaaaggaatccttatcagacaagtcaaatagatgctgcttctcccgggagaagggataggagagtctcttcatggtctggggcctgtgctcagccactttgggctggatgggatctgtgattttctggagcacagagttgatttttttcaggaggccacgggtctcattaatgtggtacatcttcttcgtcggcatcttcagtttcagaaactcggcctctctgcacagcacgttccagggggcatggattttcacaaacccgactccgtggattttagtgtcctcgtcccgctccagctccaggcccgcctccaggaggttgccctcgtactcctccctgcggaagcgcttgtcatcctcgtggtagtccatcgggggctcccccgagcctgcatccagcgacgcccccttgcccggcagggggtggtcctgcttgacgctgcgagccccagagggggtgtcgctgtgctgcaccctcctgaccagggtccggttgcccgagggcctcttgtgatggtacaccaggatgtagtccaccttgcgccggccgtccctgaagtacaggccatacttgcactcggcatcagggtccacagataaggagttcagcagcacctgggagggcctggtcagcatctggtgccggcaggaggctgaaactaagcaactgacttctctctacagtaacacagggccccgctgtgctggtgaccttcaggaggacctggactcagtgtgcgt

SEQ ID NO: 16529 - RNA, 4070 nt, Homo sapiens
  source 1..4070: mol_type = other RNA
gtgggcgggggcaggtgtgtggctgacagtggggagcctgctggggacgccaagggtgctgtttcctgcttaatcagggacacctctgtccccttctagctttccagggataactgggatgctcccacgccccctgtgtggctcagggatgaggcacttctctctcagccactcaactgatggaaggaaaaggcgatggaaagtctaacttttctgaaacaggtaggtgacaccttttggaaccggaatcaatcattattcttgcgtgggttttccattttccctgaagcatcgcaccagcttttgcgcgatgcctcggcttaccattttgcatctatcttaaggaattaggaggattcagaggagggtttctacgggcctctgctcacttttcacctctagggagactcaagtttccaagcattctttctgcaaagcacctgcctttgctaccttattgccgtattaccagccatcattttgattcatcttgaatactacagattaaaaaatattccctgcataatggctttgtgcaaaaacaagggaaagaaaacagaaagaagaaaggaaaatgtcctatcagaaagtggtcctccatgtttgcagaaaacccaggacccaccgggccctggtgggagcgggaagccgcctgccctgggagagggtgcccatcggtcaggatgcccggctggcctgcccagccccgctggcatagctacaggacgcccccgtggtaggcatggctgggggctgggctgccgaggctgtctgggcaggctttggtgttgtggtggttgcacggcggctcgtccttctgccgctccttctccatccaggtttccagcagctgctgcttgtcttgctcctcccgcatgaacagctccaccatgagcaccttctccttgtggatctgctggctgatgtccttggggatgtccgggatgacccagtccacaaagtcgctcatgaacatgaccaggttctggaagacgatgacaaacgccagccgggctgccaggacggcccagaagtccttggagatgtcgtacttgttttccgaccacggcggctctcggtagtctttatacctgcagatctgcacctcgtagcccaggtccagggggtcattgggggccgtgccgttctggaagtcactgacgttgaaggaggagagggtgtggttgacgaagccgtgcatggtcccgttcttactgtacatgtagaggtacaccaggcgcgggatgaagtcagacgtgaaggagatcacgaaggcattgatgatgacagcaagcttcccaatgcctctgaggatattgtaccagattccgatgtctttggctctgacagctaccggccttcggagctcagtgacaaactttttggcgtccaggcggatctcgatgatgttgttcagcagcgcaaacagtggggccagggggaaggaggcgacaaacagggtgacgaagccaaactggatgatcatttccatgtactctggggtgaggcccgcgaagggctccaggttgtaatccacctcgtaccgctgtttcctcttcacacactcctcgtggtcaggggggctctgctgcttcagcttcaggtagcggatgagcttcttcatcttcgggatgccgatctcgaacaggttgttctggatcagctgtttccccagcatgatgatgctgagctggatgcatagctccatcaggcagccccctggcgcacactcttccattcggaaggaacggaaaatgtacacgtagtcgcccgggcgtccaacaaaccggcctttgaagaacgccacgtaaaagatgggggtgtaggaattcacaaacttcagcaggaaagccttgaagatcagcctctcctcaaagcttttctccgtctttgggacctcgatcttggtgagccatcgggctatgcagccatacacctcgtccaggaggatgatgaccactaggttgatgatgactgcggtggctgtgactgtgacccggatgttggaccgcacggagggggaggagttcatggccaaggcggcggccatggagattctgtagatgatgacgccgaggacgatggcaaacgtcactgcaatcatgaagatgatggagaccaagttagtgaggtaggctgggaaccgatctctccatgtcagcttcactttgtcagtcaatttcacccccgccatggctgtcttaaccctctgcttccatttgtttgttgactcctctggaatatgccggcgcttctctttgtttctggactctttcttcagagacttctccaagactctggcttcgtattcagctctaggatgatccttgacagcctcctcttcctcttcaaagcccgtgaggtcccagcggtagttgagtcgcatctgtttccgcttccagtgctccatgaaggtggcagcccagagggccatgaagacagagaagaagaccgtggcggggttgtcgaagaggtggctggcgcgggccgtggcgcaggctgagctcatcttccagtagctgcaggtcttgtcgcaaagcgggcacatggtgatattgtgtctctggtcacacatctccatgctggggatgttttcatccatggtggcgcatccgtacaggaagacaatgattcccacgatggaggcagggatgagcatctgggtgtacacgcccagccaggcgaagtacaggccgatcttctccccaaaatacttcctgaccaggtcgatgggctggtacttatagaaaactccatagcgtgcccactcttcgtacaggagttttctgtcgttgaactcgacgttttcaccgttgtagtctccatcgtgcagtgggtatgcagccgcgtacacaccattggccagcaggctcgtgatgccatacttcccacatttccgccttttacttagaagggcggagtccttctttcttccctcgccttgccccatgctgtacttggcctttgtacacgtcgttctcttcaagatctcatagacaatcgtgctccgggttttgctgtcgaaaaaggaatccttatcagacaagtcaaatagatgctgcttctcccgggagaagggataggagagtctcttcatggtctggggcctgtgctcagccactttgggctggatgggatctgtgattttctggagcacagagttgatttttttcaggaggccacgggtctcattaatgtggtacatcttcttcgtcggcatcttcagtttcagaaactcggcctctctgcacagcacgttccagggggcatggattttcacaaacccgactccgtggattttagtgtcctcgtcccgctccagctccaggcccgcctccaggaggttgccctcgtactcctccctgcggaagcgcttgtcatcctcgtggtagtccatcgggggctcccccgagcctgcatccagcgacgcccccttgcccggcagggggtggtcctgcttgacgctgcgagccccagagggggtgtcgctgtgctgcaccctcctgaccagggtccggttgcccgagggcctcttgtgatggtacaccaggatgtagtccaccttgcgccggccgtccctgaagtacaggccatacttgcactcggcatcagggtccacagataaggagttcagcagcgtgccctcggacggcaggtagccgatgtcctcgatggcgcagatgttgatgatgtggacgctgcggtcctcggccgggagcgtcgagtacttctcgttgaccctcatcgtggccgcctgtgcgctgggaccgccgggcggcgcgccctccccatccacggccccggcggcctcgactgtggggacttccctggggggcagcccctccaggccgatgtcgccctcctgcatggcgcgttcgctgcgcgactccggtgcacccgggacctagcgagtccagactagggagcgacgaagtcacccctggaggtctgcggcggctctgggggccaaggtccgagcctagctcgggaggggactgtcccctctctcctccccagaggcaggagcgaagccgcgcgtgctgtagccaaacttggctgccctcgctcac

SEQ ID NO: 16530 - RNA, 3673 nt, Homo sapiens
  source 1..3673: mol_type = other RNA
gtgggcgggggcaggtgtgtggctgacagtggggagcctgctggggacgccaagggtgctgtttcctgcttaatcagggacacctctgtccccttctagctttccagggataactgggatgctcccacgccccctgtgtggctcagggatgaggcacttctctctcagccactcaactgatggaaggaaaaggcgatggaaagtctaacttttctgaaacaggtaggtgacaccttttggaaccggaatcaatcattattcttgcgtgggttttccattttccctgaagcatcgcaccagcttttgcgcgatgcctcggcttaccattttgcatctatcttaaggaattaggaggattcagaggagggtttctacgggcctctgctcacttttcacctctagggagactcaagtttccaagcattctttctgcaaagcacctgcctttgctaccttattgccgtattaccagccatcattttgattcatcttgaatactacagattaaaaaatattccctgcataatggctttgtgcaaaaacaagggaaagaaaacagaaagaagaaaggaaaatgtcctatcagaaagtggtcctccatgtttgcagaaaacccaggacccaccgggccctggtgggagcgggaagccgcctgccctgggagagggtgcccatcggtcaggatgcccggctggcctgcccagccccgctggcatagctacaggacgcccccgtggtaggcatggctgggggctgggctgccgaggctgtctgggcaggctttggtgttgtggtggttgcacggcggctcgtccttctgccgctccttctccatccaggtttccagcagctgctgcttgtcttgctcctcccgcatgaacagctccaccatgagcaccttctccttgtggatctgctggctgatgtccttggggatgtccgggatgacccagtccacaaagtcgctcatgaacatgaccaggttctggaagacgatgacaaacgccagccgggctgccaggacggcccagaagtccttggagatgtcgtacttgttttccgaccacggcggctctcggtagtctttatacctgcagatctgcacctcgtagcccaggtccagggggtcattgggggccgtgccgttctggaagtcactgacgttgaaggaggagagggtgtggttgacgaagccgtgcatggtcccgttcttactgtacatgtagaggtacaccaggcgcgggatgaagtcagacgtgaaggagatcacgaaggcattgatgatgacagcaagcttcccaatgcctctgaggatattgtaccagattccgatgtctttggctctgacagctaccggccttcggagctcagtgacaaactttttggcgtccaggcggatctcgatgatgttgttcagcagcgcaaacagtggggccagggggaaggaggcgacaaacagggtgacgaagccaaactggatgatcatttccatgtactctggggtgaggcccgcgaagggctccaggttgtaatccacctcgtaccgctgtttcctcttcacacactcctcgtggtcaggggggctctgctgcttcagcttcaggtagcggatgagcttcttcatcttcgggatgccgatctcgaacaggttgttctggatcagctgtttccccagcatgatgatgctgagctggatgcatagctccatcaggcagccccctggcgcacactcttccattcggaaggaacggaaaatgtacacgtagtcgcccgggcgtccaacaaaccggcctttgaagaacgccacgtaaaagatgggggtgtaggaattcacaaacttcagcaggaaagccttgaagatcagcctctcctcaaagcttttctccgtctttgggacctcgatcttggtgagccatcgggctatgcagccatacacctcgtccaggaggatgatgaccactaggttgatgatgactgcggtggctgtgactgtgacccggatgttggaccgcacggagggggaggagttcatggccaaggcggcggccatggagattctgtagatgatgacgccgaggacgatggcaaacgtcactgcaatcatgaagatgatggagaccaagttagtgaggtaggctgggaaccgatctctccatgtcagcttcactttgtcagtcaatttcacccccgccatggctgtcttaaccctctgcttccatttgtttgttgactcctctggaatatgccggcgcttctctttgtttctggactctttcttcagagacttctccaagactctggcttcgtattcagctctaggatgatccttgacagcctcctcttcctcttcaaagcccgtgaggtcccagcggtagttgagtcgcatctgtttccgcttccagtgctccatgaaggtggcagcccagagggccatgaagacagagaagaagaccgtggcggggttgtcgaagaggtggctggcgcgggccgtggcgcaggctgagctcatcttccagtagctgcaggtcttgtcgcaaagcgggcacatggtgatattgtgtctctggtcacacatctccatgctggggatgttttcatccatggtggcgcatccgtacaggaagacaatgattcccacgatggaggcagggatgagcatctgggtgtacacgcccagccaggcgaagtacaggccgatcttctccccaaaatacttcctgaccaggtcgatgggctggtacttatagaaaactccatagcgtgcccactcttcgtacaggagttttctgtcgttgaactcgacgttttcaccgttgtagtctccatcgtgcagtgggtatgcagccgcgtacacaccattggccagcaggctcgtgatgccatacttcccacatttccgccttttacttagaagggcggagtccttctttcttccctcgccttgccccatgctgtacttggcctttgtacacgtcgttctcttcaagatctcatagacaatcgtgctccgggttttgctgtcgaaaaaggaatccttatcagacaagtcaaatagatgctgcttctcccgggagaagggataggagagtctcttcatggtctggggcctgtgctcagccactttgggctggatgggatctgtgattttctggagcacagagttgatttttttcaggaggccacgggtctcattaatgtggtacatcttcttcgtcggcatcttcagtttcagaaactcggcctctctgcacagcacgttccagggggcatggattttcacaaacccgactccgtggattttagtgtcctcgtcccgctccagctccaggcccgcctccaggaggttgccctcgtactcctccctgcggaagcgcttgtcatcctcgtggtagtccatcgggggctcccccgagcctgcatccagcgacgcccccttgcccggcagggggtggtcctgcttgacgctgcgagccccagagggggtgtcgctgtgctgcaccctcctgaccagggtccggttgcccgagggcctcttgtgatggtacaccaggatgtagtccaccttgcgccggccgtccctgaagtacaggccatacttgcactcggcatcagggtccacagataaggagttcagcagctgggagggcctggtcagcatctggtgccggcagga

SEQ ID NO: 16531 - RNA, 3881 nt, Homo sapiens
  source 1..3881: mol_type = other RNA
gtgggcgggggcaggtgtgtggctgacagtggggagcctgctggggacgccaagggtgctgtttcctgcttaatcagggacacctctgtccccttctagctttccagggataactgggatgctcccacgccccctgtgtggctcagggatgaggcacttctctctcagccactcaactgatggaaggaaaaggcgatggaaagtctaacttttctgaaacaggtaggtgacaccttttggaaccggaatcaatcattattcttgcgtgggttttccattttccctgaagcatcgcaccagcttttgcgcgatgcctcggcttaccattttgcatctatcttaaggaattaggaggattcagaggagggtttctacgggcctctgctcacttttcacctctagggagactcaagtttccaagcattctttctgcaaagcacctgcctttgctaccttattgccgtattaccagccatcattttgattcatcttgaatactacagattaaaaaatattccctgcataatggctttgtgcaaaaacaagggaaagaaaacagaaagaagaaaggaaaatgtcctatcagaaagtggtcctccatgtttgcagaaaacccaggacccaccgggccctggtgggagcgggaagccgcctgccctgggagagggtgcccatcggtcaggatgcccggctggcctgcccagccccgctggcatagctacaggacgcccccgtggtaggcatggctgggggctgggctgccgaggctgtctgggcaggctttggtgttgtggtggttgcacggcggctcgtccttctgccgctccttctccatccaggtttccagcagctgctgcttgtcttgctcctcccgcatgaacagctccaccatgagcaccttctccttgtggatctgctggctgatgtccttggggatgtccgggatgacccagtccacaaagtcgctcatgaacatgaccaggttctggaagacgatgacaaacgccagccgggctgccaggacggcccagaagtccttggagatgtcgtacttgttttccgaccacggcggctctcggtagtctttatacctgcagatctgcacctcgtagcccaggtccagggggtcattgggggccgtgccgttctggaagtcactgacgttgaaggaggagagggtgtggttgacgaagccgtgcatggtcccgttcttactgtacatgtagaggtacaccaggcgcgggatgaagtcagacgtgaaggagatcacgaaggcattgatgatgacagcaagcttcccaatgcctctgaggatattgtaccagattccgatgtctttggctctgacagctaccggccttcggagctcagtgacaaactttttggcgtccaggcggatctcgatgatgttgttcagcagcgcaaacagtggggccagggggaaggaggcgacaaacagggtgacgaagccaaactggatgatcatttccatgtactctggggtgaggcccgcgaagggctccaggttgtaatccacctcgtaccgctgtttcctcttcacacactcctcgtggtcaggggggctctgctgcttcagcttcaggtagcggatgagcttcttcatcttcgggatgccgatctcgaacaggttgttctggatcagctgtttccccagcatgatgatgctgagctggatgcatagctccatcaggcagccccctggcgcacactcttccattcggaaggaacggaaaatgtacacgtagtcgcccgggcgtccaacaaaccggcctttgaagaacgccacgtaaaagatgggggtgtaggaattcacaaacttcagcaggaaagccttgaagatcagcctctcctcaaagcttttctccgtctttgggacctcgatcttggtgagccatcgggctatgcagccatacacctcgtccaggaggatgatgaccactaggttgatgatgactgcggtggctgtgactgtgacccggatgttggaccgcacggagggggaggagttcatggccaaggcggcggccatggagattctgtagatgatgacgccgaggacgatggcaaacgtcactgcaatcatgaagatgatggagaccaagttagtgaggtaggctgggaaccgatctctccatgtcagcttcactttgtcagtcaatttcacccccgccatggctgtcttaaccctctgcttccatttgtttgttgactcctctggaatatgccggcgcttctctttgtttctggactctttcttcagagacttctccaagactctggcttcgtattcagctctaggatgatccttgacagcctcctcttcctcttcaaagcccgtgaggtcccagcggtagttgagtcgcatctgtttccgcttccagtgctccatgaaggtggcagcccagagggccatgaagacagagaagaagaccgtggcggggttgtcgaagaggtggctggcgcgggccgtggcgcaggctgagctcatcttccagtagctgcaggtcttgtcgcaaagcgggcacatggtgatattgtgtctctggtcacacatctccatgctggggatgttttcatccatggtggcgcatccgtacaggaagacaatgattcccacgatggaggcagggatgagcatctgggtgtacacgcccagccaggcgaagtacaggccgatcttctccccaaaatacttcctgaccaggtcgatgggctggtacttatagaaaactccatagcgtgcccactcttcgtacaggagttttctgtcgttgaactcgacgttttcaccgttgtagtctccatcgtgcagtgggtatgcagccgcgtacacaccattggccagcaggctcgtgatgccatacttcccacatttccgccttttacttagaagggcggagtccttctttcttccctcgccttgccccatgctgtacttggcctttgtacacgtcgttctcttcaagatctcatagacaatcgtgctccgggttttgctgtcgaaaaaggaatccttatcagacaagtcaaatagatgctgcttctcccgggagaagggataggagagtctcttcatggtctggggcctgtgctcagccactttgggctggatgggatctgtgattttctggagcacagagttgatttttttcaggaggccacgggtctcattaatgtggtacatcttcttcgtcggcatcttcagtttcagaaactcggcctctctgcacagcacgttccagggggcatggattttcacaaacccgactccgtggattttagtgtcctcgtcccgctccagctccaggcccgcctccaggaggttgccctcgtactcctccctgcggaagcgcttgtcatcctcgtggtagtccatcgggggctcccccgagcctgcatccagcgacgcccccttgcccggcagggggtggtcctgcttgacgctgcgagccccagagggggtgtcgctgtgctgcaccctcctgaccagggtccggttgcccgagggcctcttgtgatggtacaccaggatgtagtccaccttgcgccggccgtccctgaagtacaggccatacttgcactcggcatcagggtccacagataaggagttcagcagctttcataggtgttgatgtcaagggtctagactcctctacccctggttaggggacagttggggccatgtccctggcaccttggcctctctggccctaggatgcctctcctggaaacagcattgctcaccacctgggagggcctggtcagcatctggtgccggcaggaggctgaaactaagcaactgacttctctctacagtaacacagggccccgctgtgctggtgaccttcaggaggacctgg

SEQ ID NO: 16532 - RNA, 3746 nt, Homo sapiens
  source 1..3746: mol_type = other RNA
gtgggcgggggcaggtgtgtggctgacagtggggagcctgctggggacgccaagggtgctgtttcctgcttaatcagggacacctctgtccccttctagctttccagggataactgggatgctcccacgccccctgtgtggctcagggatgaggcacttctctctcagccactcaactgatggaaggaaaaggcgatggaaagtctaacttttctgaaacaggtaggtgacaccttttggaaccggaatcaatcattattcttgcgtgggttttccattttccctgaagcatcgcaccagcttttgcgcgatgcctcggcttaccattttgcatctatcttaaggaattaggaggattcagaggagggtttctacgggcctctgctcacttttcacctctagggagactcaagtttccaagcattctttctgcaaagcacctgcctttgctaccttattgccgtattaccagccatcattttgattcatcttgaatactacagattaaaaaatattccctgcataatggctttgtgcaaaaacaagggaaagaaaacagaaagaagaaaggaaaatgtcctatcagaaagtggtcctccatgtttgcagaaaacccaggacccaccgggccctggtgggagcgggaagccgcctgccctgggagagggtgcccatcggtcaggatgcccggctggcctgcccagccccgctggcatagctacaggacgcccccgtggtaggcatggctgggggctgggctgccgaggctgtctgggcaggctttggtgttgtggtggttgcacggcggctcgtccttctgccgctccttctccatccaggtttccagcagctgctgcttgtcttgctcctcccgcatgaacagctccaccatgagcaccttctccttgtggatctgctggctgatgtccttggggatgtccgggatgacccagtccacaaagtcgctcatgaacatgaccaggttctggaagacgatgacaaacgccagccgggctgccaggacggcccagaagtccttggagatgtcgtacttgttttccgaccacggcggctctcggtagtctttatacctgcagatctgcacctcgtagcccaggtccagggggtcattgggggccgtgccgttctggaagtcactgacgttgaaggaggagagggtgtggttgacgaagccgtgcatggtcccgttcttactgtacatgtagaggtacaccaggcgcgggatgaagtcagacgtgaaggagatcacgaaggcattgatgatgacagcaagcttcccaatgcctctgaggatattgtaccagattccgatgtctttggctctgacagctaccggccttcggagctcagtgacaaactttttggcgtccaggcggatctcgatgatgttgttcagcagcgcaaacagtggggccagggggaaggaggcgacaaacagggtgacgaagccaaactggatgatcatttccatgtactctggggtgaggcccgcgaagggctccaggttgtaatccacctcgtaccgctgtttcctcttcacacactcctcgtggtcaggggggctctgctgcttcagcttcaggtagcggatgagcttcttcatcttcgggatgccgatctcgaacaggttgttctggatcagctgtttccccagcatgatgatgctgagctggatgcatagctccatcaggcagccccctggcgcacactcttccattcggaaggaacggaaaatgtacacgtagtcgcccgggcgtccaacaaaccggcctttgaagaacgccacgtaaaagatgggggtgtaggaattcacaaacttcagcaggaaagccttgaagatcagcctctcctcaaagcttttctccgtctttgggacctcgatcttggtgagccatcgggctatgcagccatacacctcgtccaggaggatgatgaccactaggttgatgatgactgcggtggctgtgactgtgacccggatgttggaccgcacggagggggaggagttcatggccaaggcggcggccatggagattctgtagatgatgacgccgaggacgatggcaaacgtcactgcaatcatgaagatgatggagaccaagttagtgaggtaggctgggaaccgatctctccatgtcagcttcactttgtcagtcaatttcacccccgccatggctgtcttaaccctctgcttccatttgtttgttgactcctctggaatatgccggcgcttctctttgtttctggactctttcttcagagacttctccaagactctggcttcgtattcagctctaggatgatccttgacagcctcctcttcctcttcaaagcccgtgaggtcccagcggtagttgagtcgcatctgtttccgcttccagtgctccatgaaggtggcagcccagagggccatgaagacagagaagaagaccgtggcggggttgtcgaagaggtggctggcgcgggccgtggcgcaggctgagctcatcttccagtagctgcaggtcttgtcgcaaagcgggcacatggtgatattgtgtctctggtcacacatctccatgctggggatgttttcatccatggtggcgcatccgtacaggaagacaatgattcccacgatggaggcagggatgagcatctgggtgtacacgcccagccaggcgaagtacaggccgatcttctccccaaaatacttcctgaccaggtcgatgggctggtacttatagaaaactccatagcgtgcccactcttcgtacaggagttttctgtcgttgaactcgacgttttcaccgttgtagtctccatcgtgcagtgggtatgcagccgcgtacacaccattggccagcaggctcgtgatgcccatgctgtacttggcctttgtacacgtcgttctcttcaagatctcatagacaatcgtgctccgggttttgctgtcgaaaaaggaatccttatcagacaagtcaaatagatgctgcttctcccgggagaagggataggagagtctcttcatggtctggggcctgtgctcagccactttgggctggatgggatctgtgattttctggagcacagagttgatttttttcaggaggccacgggtctcattaatgtggtacatcttcttcgtcggcatcttcagtttcagaaactcggcctctctgcacagcacgttccagggggcatggattttcacaaacccgactccgtggattttagtgtcctcgtcccgctccagctccaggcccgcctccaggaggttgccctcgtactcctccctgcggaagcgcttgtcatcctcgtggtagtccatcgggggctcccccgagcctgcatccagcgacgcccccttgcccggcagggggtggtcctgcttgacgctgcgagccccagagggggtgtcgctgtgctgcaccctcctgaccagggtccggttgcccgagggcctcttgtgatggtacaccaggatgtagtccaccttgcgccggccgtccctgaagtacaggccatacttgcactcggcatcagggtccacagataaggagttcagcagcgtgccctcggacggcaggtagccgatgtcctcgatggcgcagatgttgatgatgtggacgctgcggtcctcggccgggagcgtcgagtacttctcgttgaccctcatcgtggccgcctgtgcgctgggaccgccgggcggcgcgccctccccatccacggccccggcggcctct

SEQ ID NO: 16533 - RNA, 3755 nt, Homo sapiens
  source 1..3755: mol_type = other RNA
gtgggcgggggcaggtgtgtggctgacagtggggagcctgctggggacgccaagggtgctgtttcctgcttaatcagggacacctctgtccccttctagctttccagggataactgggatgctcccacgccccctgtgtggctcagggatgaggcacttctctctcagccactcaactgatggaaggaaaaggcgatggaaagtctaacttttctgaaacaggtaggtgacaccttttggaaccggaatcaatcattattcttgcgtgggttttccattttccctgaagcatcgcaccagcttttgcgcgatgcctcggcttaccattttgcatctatcttaaggaattaggaggattcagaggagggtttctacgggcctctgctcacttttcacctctagggagactcaagtttccaagcattctttctgcaaagcacctgcctttgctaccttattgccgtattaccagccatcattttgattcatcttgaatactacagattaaaaaatattccctgcataatggctttgtgcaaaaacaagggaaagaaaacagaaagaagaaaggaaaatgtcctatcagaaagtggtcctccatgtttgcagaaaacccaggacccaccgggccctggtgggagcgggaagccgcctgccctgggagagggtgcccatcggtcaggatgcccggctggcctgcccagccccgctggcatagctacaggacgcccccgtggtaggcatggctgggggctgggctgccgaggctgtctgggcaggctttggtgttgtggtggttgcacggcggctcgtccttctgccgctccttctccatccaggtttccagcagctgctgcttgtcttgctcctcccgcatgaacagctccaccatgagcaccttctccttgtggatctgctggctgatgtccttggggatgtccgggatgacccagtccacaaagtcgctcatgaacatgaccaggttctggaagacgatgacaaacgccagccgggctgccaggacggcccagaagtccttggagatgtcgtacttgttttccgaccacggcggctctcggtagtctttatacctgcagatctgcacctcgtagcccaggtccagggggtcattgggggccgtgccgttctggaagtcactgacgttgaaggaggagagggtgtggttgacgaagccgtgcatggtcccgttcttactgtacatgtagaggtacaccaggcgcgggatgaagtcagacgtgaaggagatcacgaaggcattgatgatgacagcaagcttcccaatgcctctgaggatattgtaccagattccgatgtctttggctctgacagctaccggccttcggagctcagtgacaaactttttggcgtccaggcggatctcgatgatgttgttcagcagcgcaaacagtggggccagggggaaggaggcgacaaacagggtgacgaagccaaactggatgatcatttccatgtactctggggtgaggcccgcgaagggctccaggttgtaatccacctcgtaccgctgtttcctcttcacacactcctcgtggtcaggggggctctgctgcttcagcttcaggtagcggatgagcttcttcatcttcgggatgccgatctcgaacaggttgttctggatcagctgtttccccagcatgatgatgctgagctggatgcatagctccatcaggcagccccctggcgcacactcttccattcggaaggaacggaaaatgtacacgtagtcgcccgggcgtccaacaaaccggcctttgaagaacgccacgtaaaagatgggggtgtaggaattcacaaacttcagcaggaaagccttgaagatcagcctctcctcaaagcttttctccgtctttgggacctcgatcttggtgagccatcgggctatgcagccatacacctcgtccaggaggatgatgaccactaggttgatgatgactgcggtggctgtgactgtgacccggatgttggaccgcacggagggggaggagttcatggccaaggcggcggccatggagattctgtagatgatgacgccgaggacgatggcaaacgtcactgcaatcatgaagatgatggagaccaagttagtgaggtaggctgggaaccgatctctccatgtcagcttcactttgtcagtcaatttcacccccgccatggctgtcttaaccctctgcttccatttgtttgttgactcctctggaatatgccggcgcttctctttgtttctggactctttcttcagagacttctccaagactctggcttcgtattcagctctaggatgatccttgacagcctcttcctcttcaaagcccgtgaggtcccagcggtagttgagtcgcatctgtttccgcttccagtgctccatgaaggtggcagcccagagggccatgaagacagagaagaagaccgtggcggggttgtcgaagaggtggctggcgcgggccgtggcgcaggctgagctcatcttccagtagctgcaggtcttgtcgcaaagcgggcacatggtgatattgtgtctctggtcacacatctccatgctggggatgttttcatccatggtggcgcatccgtacaggaagacaatgattcccacgatggaggcagggatgagcatctgggtgtacacgcccagccaggcgaagtacaggccgatcttctccccaaaatacttcctgaccaggtcgatgggctggtacttatagaaaactccatagcgtgcccactcttcgtacaggagttttctgtcgttgaactcgacgttttcaccgttgtagtctccatcgtgcagtgggtatgcagccgcgtacacaccattggccagcaggctcgtgatgccatacttcccacatttccgccttttacttagaagggcggagtccttctttcttccctcgccttgccccatgctgtacttggcctttgtacacgtcgttctcttcaagatctcatagacaatcgtgctccgggttttgctgtcgaaaaaggaatccttatcagacaagtcaaatagatgctgcttctcccgggagaagggataggagagtctcttcatggtctggggcctgtgctcagccactttgggctggatgggatctgtgattttctggagcacagagttgatttttttcaggaggccacgggtctcattaatgtggtacatcttcttcgtcggcatcttcagtttcagaaactcggcctctctgcacagcacgttccagggggcatggattttcacaaacccgactccgtggattttagtgtcctcgtcccgctccagctccaggcccgcctccaggaggttgccctcgtactcctccctgcggaagcgcttgtcatcctcgtggtagtccatcgggggctcccccgagcctgcatccagcgacgcccccttgcccggcagggggtggtcctgcttgacgctgcgagccccagagggggtgtcgctgtgctgcaccctcctgaccagggtccggttgcccgagggcctcttgtgatggtacaccaggatgtagtccaccttgcgccggccgtccctgaagtacaggccatacttgcactcggcatcagggtccacagataaggagttcagcagcgtgccctcggacggcaggtagccgatgtcctcgatggcgcagatgttgatgatgtggacgctgcggtcctcggccgggagcgtcgagtacttctcgttgaccctcatcgtggccgcctgt

SEQ ID NO: 16534 - RNA, 3689 nt, Homo sapiens
  source 1..3689: mol_type = other RNA
gtgggcgggggcaggtgtgtggctgacagtggggagcctgctggggacgccaagggtgctgtttcctgcttaatcagggacacctctgtccccttctagctttccagggataactgggatgctcccacgccccctgtgtggctcagggatgaggcacttctctctcagccactcaactgatggaaggaaaaggcgatggaaagtctaacttttctgaaacaggtaggtgacaccttttggaaccggaatcaatcattattcttgcgtgggttttccattttccctgaagcatcgcaccagcttttgcgcgatgcctcggcttaccattttgcatctatcttaaggaattaggaggattcagaggagggtttctacgggcctctgctcacttttcacctctagggagactcaagtttccaagcattctttctgcaaagcacctgcctttgctaccttattgccgtattaccagccatcattttgattcatcttgaatactacagattaaaaaatattccctgcataatggctttgtgcaaaaacaagggaaagaaaacagaaagaagaaaggaaaatgtcctatcagaaagtggtcctccatgtttgcagaaaacccaggacccaccgggccctggtgggagcgggaagccgcctgccctgggagagggtgcccatcggtcaggatgcccggctggcctgcccagccccgctggcatagctacaggacgcccccgtggtaggcatggctgggggctgggctgccgaggctgtctgggcaggctttggtgttgtggtggttgcacggcggctcgtccttctgccgctccttctccatccaggtttccagcagctgctgcttgtcttgctcctcccgcatgaacagctccaccatgagcaccttctccttgtggatctgctggctgatgtccttggggatgtccgggatgacccagtccacaaagtcgctcatgaacatgaccaggttctggaagacgatgacaaacgccagccgggctgccaggacggcccagaagtccttggagatgtcgtacttgttttccgaccacggcggctctcggtagtctttatacctgcagatctgcacctcgtagcccaggtccagggggtcattgggggccgtgccgttctggaagtcactgacgttgaaggaggagagggtgtggttgacgaagccgtgcatggtcccgttcttactgtacatgtagaggtacaccaggcgcgggatgaagtcagacgtgaaggagatcacgaaggcattgatgatgacagcaagcttcccaatgcctctgaggatattgtaccagattccgatgtctttggctctgacagctaccggccttcggagctcagtgacaaactttttggcgtccaggcggatctcgatgatgttgttcagcagcgcaaacagtggggccagggggaaggaggcgacaaacagggtgacgaagccaaactggatgatcatttccatgtactctggggtgaggcccgcgaagggctccaggttgtaatccacctcgtaccgctgtttcctcttcacacactcctcgtggtcaggggggctctgctgcttcagcttcaggtagcggatgagcttcttcatcttcgggatgccgatctcgaacaggttgttctggatcagctgtttccccagcatgatgatgctgagctggatgcatagctccatcaggcagccccctggcgcacactcttccattcggaaggaacggaaaatgtacacgtagtcgcccgggcgtccaacaaaccggcctttgaagaacgccacgtaaaagatgggggtgtaggaattcacaaacttcagcaggaaagccttgaagatcagcctctcctcaaagcttttctccgtctttgggacctcgatcttggtgagccatcgggctatgcagccatacacctcgtccaggaggatgatgaccactaggttgatgatgactgcggtggctgtgactgtgacccggatgttggaccgcacggagggggaggagttcatggccaaggcggcggccatggagattctgtagatgatgacgccgaggacgatggcaaacgtcactgcaatcatgaagatgatggagaccaagttagtgaggtaggctgggaaccgatctctccatgtcagcttcactttgtcagtcaatttcacccccgccatggctgtcttaaccctctgcttccatttgtttgttgactcctctggaatatgccggcgcttctctttgtttctggactctttcttcagagacttctccaagactctggcttcgtattcagctctaggatgatccttgacagcctcttcctcttcaaagcccgtgaggtcccagcggtagttgagtcgcatctgtttccgcttccagtgctccatgaaggtggcagcccagagggccatgaagacagagaagaagaccgtggcggggttgtcgaagaggtggctggcgcgggccgtggcgcaggctgagctcatcttccagtagctgcaggtcttgtcgcaaagcgggcacatggtgatattgtgtctctggtcacacatctccatgctggggatgttttcatccatggtggcgcatccgtacaggaagacaatgattcccacgatggaggcagggatgagcatctgggtgtacacgcccagccaggcgaagtacaggccgatcttctccccaaaatacttcctgaccaggtcgatgggctggtacttatagaaaactccatagcgtgcccactcttcgtacaggagttttctgtcgttgaactcgacgttttcaccgttgtagtctccatcgtgcagtgggtatgcagccgcgtacacaccattggccagcaggctcgtgatgcccatgctgtacttggcctttgtacacgtcgttctcttcaagatctcatagacaatcgtgctccgggttttgctgtcgaaaaaggaatccttatcagacaagtcaaatagatgctgcttctcccgggagaagggataggagagtctcttcatggtctggggcctgtgctcagccactttgggctggatgggatctgtgattttctggagcacagagttgatttttttcaggaggccacgggtctcattaatgtggtacatcttcttcgtcggcatcttcagtttcagaaactcggcctctctgcacagcacgttccagggggcatggattttcacaaacccgactccgtggattttagtgtcctcgtcccgctccagctccaggcccgcctccaggaggttgccctcgtactcctccctgcggaagcgcttgtcatcctcgtggtagtccatcgggggctcccccgagcctgcatccagcgacgcccccttgcccggcagggggtggtcctgcttgacgctgcgagccccagagggggtgtcgctgtgctgcaccctcctgaccagggtccggttgcccgagggcctcttgtgatggtacaccaggatgtagtccaccttgcgccggccgtccctgaagtacaggccatacttgcactcggcatcagggtccacagataaggagttcagcagcgtgccctcggacggcaggtagccgatgtcctcgatggcgcagatgttgatgatgtggacgctgcggtcctcggccgggagcgtcgagtacttctcgttgaccctcatcgtggccgcctgt

SEQ ID NO: 16535 - RNA, 3668 nt, Homo sapiens
  source 1..3668: mol_type = other RNA
gtgggcgggggcaggtgtgtggctgacagtggggagcctgctggggacgccaagggtgctgtttcctgcttaatcagggacacctctgtccccttctagctttccagggataactgggatgctcccacgccccctgtgtggctcagggatgaggcacttctctctcagccactcaactgatggaaggaaaaggcgatggaaagtctaacttttctgaaacaggtaggtgacaccttttggaaccggaatcaatcattattcttgcgtgggttttccattttccctgaagcatcgcaccagcttttgcgcgatgcctcggcttaccattttgcatctatcttaaggaattaggaggattcagaggagggtttctacgggcctctgctcacttttcacctctagggagactcaagtttccaagcattctttctgcaaagcacctgcctttgctaccttattgccgtattaccagccatcattttgattcatcttgaatactacagattaaaaaatattccctgcataatggctttgtgcaaaaacaagggaaagaaaacagaaagaagaaaggaaaatgtcctatcagaaagtggtcctccatgtttgcagaaaacccaggacccaccgggccctggtgggagcgggaagccgcctgccctgggagagggtgcccatcggtcaggatgcccggctggcctgcccagccccgctggcatagctacaggacgcccccgtggtaggcatggctgggggctgggctgccgaggctgtctgggcaggctttggtgttgtggtggttgcacggcggctcgtccttctgccgctccttctccatccaggtttccagcagctgctgcttgtcttgctcctcccgcatgaacagctccaccatgagcaccttctccttgtggatctgctggctgatgtccttggggatgtccgggatgacccagtccacaaagtcgctcatgaacatgaccaggttctggaagacgatgacaaacgccagccgggctgccaggacggcccagaagtccttggagatgtcgtacttgttttccgaccacggcggctctcggtagtctttatacctgcagatctgcacctcgtagcccaggtccagggggtcattgggggccgtgccgttctggaagtcactgacgttgaaggaggagagggtgtggttgacgaagccgtgcatggtcccgttcttactgtacatgtagaggtacaccaggcgcgggatgaagtcagacgtgaaggagatcacgaaggcattgatgatgacagcaagcttcccaatgcctctgaggatattgtaccagattccgatgtctttggctctgacagctaccggccttcggagctcagtgacaaactttttggcgtccaggcggatctcgatgatgttgttcagcagcgcaaacagtggggccagggggaaggaggcgacaaacagggtgacgaagccaaactggatgatcatttccatgtactctggggtgaggcccgcgaagggctccaggttgtaatccacctcgtaccgctgtttcctcttcacacactcctcgtggtcaggggggctctgctgcttcagcttcaggtagcggatgagcttcttcatcttcgggatgccgatctcgaacaggttgttctggatcagctgtttccccagcatgatgatgctgagctggatgcatagctccatcaggcagccccctggcgcacactcttccattcggaaggaacggaaaatgtacacgtagtcgcccgggcgtccaacaaaccggcctttgaagaacgccacgtaaaagatgggggtgtaggaattcacaaacttcagcaggaaagccttgaagatcagcctctcctcaaagcttttctccgtctttgggacctcgatcttggtgagccatcgggctatgcagccatacacctcgtccaggaggatgatgaccactaggttgatgatgactgcggtggctgtgactgtgacccggatgttggaccgcacggagggggaggagttcatggccaaggcggcggccatggagattctgtagatgatgacgccgaggacgatggcaaacgtcactgcaatcatgaagatgatggagaccaagttagtgaggtaggctgggaaccgatctctccatgtcagcttcactttgtcagtctctttgtttctggactctttcttcagagacttctccaagactctggcttcgtattcagctctaggatgatcctcttcctcttcaaagcccgtgaggtcccagcggtagttgagtcgcatctgtttccgcttccagtgctccatgaaggtggcagcccagagggccatgaagacagagaagaagaccgtggcggggttgtcgaagaggtggctggcgcgggccgtggcgcaggctgagctcatcttccagtagctgcaggtcttgtcgcaaagcgggcacatggtgatattgtgtctctggtcacacatctccatgctggggatgttttcatccatggtggcgcatccgtacaggaagacaatgattcccacgatggaggcagggatgagcatctgggtgtacacgcccagccaggcgaagtacaggccgatcttctccccaaaatacttcctgaccaggtcgatgggctggtacttatagaaaactccatagcgtgcccactcttcgtacaggagttttctgtcgttgaactcgacgttttcaccgttgtagtctccatcgtgcagtgggtatgcagccgcgtacacaccattggccagcaggctcgtgatgccatacttcccacatttccgccttttacttagaagggcggagtccttctttcttccctcgccttgccccatgctgtacttggcctttgtacacgtcgttctcttcaagatctcatagacaatcgtgctccgggttttgctgtcgaaaaaggaatccttatcagacaagtcaaatagatgctgcttctcccgggagaagggataggagagtctcttcatggtctggggcctgtgctcagccactttgggctggatgggatctgtgattttctggagcacagagttgatttttttcaggaggccacgggtctcattaatgtggtacatcttcttcgtcggcatcttcagtttcagaaactcggcctctctgcacagcacgttccagggggcatggattttcacaaacccgactccgtggattttagtgtcctcgtcccgctccagctccaggcccgcctccaggaggttgccctcgtactcctccctgcggaagcgcttgtcatcctcgtggtagtccatcgggggctcccccgagcctgcatccagcgacgcccccttgcccggcagggggtggtcctgcttgacgctgcgagccccagagggggtgtcgctgtgctgcaccctcctgaccagggtccggttgcccgagggcctcttgtgatggtacaccaggatgtagtccaccttgcgccggccgtccctgaagtacaggccatacttgcactcggcatcagggtccacagataaggagttcagcagcgtgccctcggacggcaggtagccgatgtcctcgatggcgcagatgttgatgatgtggacgctgcggtcctcggccgggagcgtcgagtacttctcgttgaccctcatcgtggccgcctgt

SEQ ID NO: 16536 - RNA, 3656 nt, Homo sapiens
  source 1..3656: mol_type = other RNA
gtgggcgggggcaggtgtgtggctgacagtggggagcctgctggggacgccaagggtgctgtttcctgcttaatcagggacacctctgtccccttctagctttccagggataactgggatgctcccacgccccctgtgtggctcagggatgaggcacttctctctcagccactcaactgatggaaggaaaaggcgatggaaagtctaacttttctgaaacaggtaggtgacaccttttggaaccggaatcaatcattattcttgcgtgggttttccattttccctgaagcatcgcaccagcttttgcgcgatgcctcggcttaccattttgcatctatcttaaggaattaggaggattcagaggagggtttctacgggcctctgctcacttttcacctctagggagactcaagtttccaagcattctttctgcaaagcacctgcctttgctaccttattgccgtattaccagccatcattttgattcatcttgaatactacagattaaaaaatattccctgcataatggctttgtgcaaaaacaagggaaagaaaacagaaagaagaaaggaaaatgtcctatcagaaagtggtcctccatgtttgcagaaaacccaggacccaccgggccctggtgggagcgggaagccgcctgccctgggagagggtgcccatcggtcaggatgcccggctggcctgcccagccccgctggcatagctacaggacgcccccgtggtaggcatggctgggggctgggctgccgaggctgtctgggcaggctttggtgttgtggtggttgcacggcggctcgtccttctgccgctccttctccatccaggtttccagcagctgctgcttgtcttgctcctcccgcatgaacagctccaccatgagcaccttctccttgtggatctgctggctgatgtccttggggatgtccgggatgacccagtccacaaagtcgctcatgaacatgaccaggttctggaagacgatgacaaacgccagccgggctgccaggacggcccagaagtccttggagatgtcgtacttgttttccgaccacggcggctctcggtagtctttatacctgcagatctgcacctcgtagcccaggtccagggggtcattgggggccgtgccgttctggaagtcactgacgttgaaggaggagagggtgtggttgacgaagccgtgcatggtcccgttcttactgtacatgtagaggtacaccaggcgcgggatgaagtcagacgtgaaggagatcacgaaggcattgatgatgacagcaagcttcccaatgcctctgaggatattgtaccagattccgatgtctttggctctgacagctaccggccttcggagctcagtgacaaactttttggcgtccaggcggatctcgatgatgttgttcagcagcgcaaacagtggggccagggggaaggaggcgacaaacagggtgacgaagccaaactggatgatcatttccatgtactctggggtgaggcccgcgaagggctccaggttgtaatccacctcgtaccgctgtttcctcttcacacactcctcgtggtcaggggggctctgctgcttcagcttcaggtagcggatgagcttcttcatcttcgggatgccgatctcgaacaggttgttctggatcagctgtttccccagcatgatgatgctgagctggatgcatagctccatcaggcagccccctggcgcacactcttccattcggaaggaacggaaaatgtacacgtagtcgcccgggcgtccaacaaaccggcctttgaagaacgccacgtaaaagatgggggtgtaggaattcacaaacttcagcaggaaagccttgaagatcagcctctcctcaaagcttttctccgtctttgggacctcgatcttggtgagccatcgggctatgcagccatacacctcgtccaggaggatgatgaccactaggttgatgatgactgcggtggctgtgactgtgacccggatgttggaccgcacggagggggaggagttcatggccaaggcggcggccatggagattctgtagatgatgacgccgaggacgatggcaaacgtcactgcaatcatgaagatgatggagaccaagttagtgaggtaggctgggaaccgatctctccatgtcagcttcactttgtcagtctctttgtttctggactctttcttcagagacttctccaagactctggcttcgtattcagctctaggatgatcctcttcctcttcaaagcccgtgaggtcccagcggtagttgagtcgcatctgtttccgcttccagtgctccatgaaggtggcagcccagagggccatgaagacagagaagaagaccgtggcggggttgtcgaagaggtggctggcgcgggccgtggcgcaggctgagctcatcttccagtagctgcaggtcttgtcgcaaagcgggcacatggtgatattgtgtctctggtcacacatctccatgctggggatgttttcatccatggtggcgcatccgtacaggaagacaatgattcccacgatggaggcagggatgagcatctgggtgtacacgcccagccaggcgaagtacaggccgatcttctccccaaaatacttcctgaccaggtcgatgggctggtacttatagaaaactccatagcgtgcccactcttcgtacaggagttttctgtcgttgaactcgacgttttcaccgttgtagtctccatcgtgcagtgggtatgcagccgcgtacacaccattggccagcaggctcgtgatgcccatgctgtacttggcctttgtacacgtcgttctcttcaagatctcatagacaatcgtgctccgggttttgctgtcgaaaaaggaatccttatcagacaagtcaaatagatgctgcttctcccgggagaagggataggagagtctcttcatggtctggggcctgtgctcagccactttgggctggatgggatctgtgattttctggagcacagagttgatttttttcaggaggccacgggtctcattaatgtggtacatcttcttcgtcggcatcttcagtttcagaaactcggcctctctgcacagcacgttccagggggcatggattttcacaaacccgactccgtggattttagtgtcctcgtcccgctccagctccaggcccgcctccaggaggttgccctcgtactcctccctgcggaagcgcttgtcatcctcgtggtagtccatcgggggctcccccgagcctgcatccagcgacgcccccttgcccggcagggggtggtcctgcttgacgctgcgagccccagagggggtgtcgctgtgctgcaccctcctgaccagggtccggttgcccgagggcctcttgtgatggtacaccaggatgtagtccaccttgcgccggccgtccctgaagtacaggccatacttgcactcggcatcagggtccacagataaggagttcagcagcgtgccctcggacggcaggtagccgatgtcctcgatggcgcagatgttgatgatgtggacgctgcggtcctcggccgggagcgtcgagtacttctcgttgaccctcatcgtggccgcctgtgcgctgggaccgccgggcggcgcgccctccccatccacggccccggcggcctct

SEQ ID NO: 16537 - RNA, 3737 nt, Homo sapiens
  source 1..3737: mol_type = other RNA
gtgggcgggggcaggtgtgtggctgacagtggggagcctgctggggacgccaagggtgctgtttcctgcttaatcagggacacctctgtccccttctagctttccagggataactgggatgctcccacgccccctgtgtggctcagggatgaggcacttctctctcagccactcaactgatggaaggaaaaggcgatggaaagtctaacttttctgaaacaggtaggtgacaccttttggaaccggaatcaatcattattcttgcgtgggttttccattttccctgaagcatcgcaccagcttttgcgcgatgcctcggcttaccattttgcatctatcttaaggaattaggaggattcagaggagggtttctacgggcctctgctcacttttcacctctagggagactcaagtttccaagcattctttctgcaaagcacctgcctttgctaccttattgccgtattaccagccatcattttgattcatcttgaatactacagattaaaaaatattccctgcataatggctttgtgcaaaaacaagggaaagaaaacagaaagaagaaaggaaaatgtcctatcagaaagtggtcctccatgtttgcagaaaacccaggacccaccgggccctggtgggagcgggaagccgcctgccctgggagagggtgcccatcggtcaggatgcccggctggcctgcccagccccgctggcatagctacaggacgcccccgtggtaggcatggctgggggctgggctgccgaggctgtctgggcaggctttggtgttgtggtggttgcacggcggctcgtccttctgccgctccttctccatccaggtttccagcagctgctgcttgtcttgctcctcccgcatgaacagctccaccatgagcaccttctccttgtggatctgctggctgatgtccttggggatgtccgggatgacccagtccacaaagtcgctcatgaacatgaccaggttctggaagacgatgacaaacgccagccgggctgccaggacggcccagaagtccttggagatgtcgtacttgttttccgaccacggcggctctcggtagtctttatacctgcagatctgcacctcgtagcccaggtccagggggtcattgggggccgtgccgttctggaagtcactgacgttgaaggaggagagggtgtggttgacgaagccgtgcatggtcccgttcttactgtacatgtagaggtacaccaggcgcgggatgaagtcagacgtgaaggagatcacgaaggcattgatgatgacagcaagcttcccaatgcctctgaggatattgtaccagattccgatgtctttggctctgacagctaccggccttcggagctcagtgacaaactttttggcgtccaggcggatctcgatgatgttgttcagcagcgcaaacagtggggccagggggaaggaggcgacaaacagggtgacgaagccaaactggatgatcatttccatgtactctggggtgaggcccgcgaagggctccaggttgtaatccacctcgtaccgctgtttcctcttcacacactcctcgtggtcaggggggctctgctgcttcagcttcaggtagcggatgagcttcttcatcttcgggatgccgatctcgaacaggttgttctggatcagctgtttccccagcatgatgatgctgagctggatgcatagctccatcaggcagccccctggcgcacactcttccattcggaaggaacggaaaatgtacacgtagtcgcccgggcgtccaacaaaccggcctttgaagaacgccacgtaaaagatgggggtgtaggaattcacaaacttcagcaggaaagccttgaagatcagcctctcctcaaagcttttctccgtctttgggacctcgatcttggtgagccatcgggctatgcagccatacacctcgtccaggaggatgatgaccactaggttgatgatgactgcggtggctgtgactgtgacccggatgttggaccgcacggagggggaggagttcatggccaaggcggcggccatggagattctgtagatgatgacgccgaggacgatggcaaacgtcactgcaatcatgaagatgatggagaccaagttagtgaggtaggctgggaaccgatctctccatgtcagcttcactttgtcagtctctttgtttctggactctttcttcagagacttctccaagactctggcttcgtattcagctctaggatgatcctcttcctcttcaaagcccgtgaggtcccagcggtagttgagtcgcatctgtttccgcttccagtgctccatgaaggtggcagcccagagggccatgaagacagagaagaagaccgtggcggggttgtcgaagaggtggctggcgcgggccgtggcgcaggctgagctcatcttccagtagctgcaggtcttgtcgcaaagcgggcacatggtgatattgtgtctctggtcacacatctccatgctggggatgttttcatccatggtggcgcatccgtacaggaagacaatgattcccacgatggaggcagggatgagcatctgggtgtacacgcccagccaggcgaagtacaggccgatcttctccccaaaatacttcctgaccaggtcgatgggctggtacttatagaaaactccatagcgtgcccactcttcgtacaggagttttctgtcgttgaactcgacgttttcaccgttgtagtctccatcgtgcagtgggtatgcagccgcgtacacaccattggccagcaggctcgtgatgcccatgctgtacttggcctttgtacacgtcgttctcttcaagatctcatagacaatcgtgctccgggttttgctgtcgaaaaaggaatccttatcagacaagtcaaatagatgctgcttctcccgggagaagggataggagagtctcttcatggtctggggcctgtgctcagccactttgggctggatgggatctgtgattttctggagcacagagttgatttttttcaggaggccacgggtctcattaatgtggtacatcttcttcgtcggcatcttcagtttcagaaactcggcctctctgcacagcacgttccagggggcatggattttcacaaacccgactccgtggattttagtgtcctcgtcccgctccagctccaggcccgcctccaggaggttgccctcgtactcctccctgcggaagcgcttgtcatcctcgtggtagtccatcgggggctcccccgagcctgcatccagcgacgcccccttgcccggcagggggtggtcctgcttgacgctgcgagccccagagggggtgtcgctgtgctgcaccctcctgaccagggtccggttgcccgagggcctcttgtgatggtacaccaggatgtagtccaccttgcgccggccgtccctgaagtacaggccatacttgcactcggcatcagggtccacagataaggagttcagcagctttcataggtgttgatgtcaagggtctagactcctctacccctggttaggggacagttggggccatgtccctggcaccttggcctctctggccctaggatgcctctcctggaaacagcattgctcaccacctgggagggcctggtcagcatctggtgccggcaggaggctgaaactaagcaactgacttctctctacagtaacacagggccccgctgtgctggtgaccttcaggaggacctggactcagtgtgcg

SEQ ID NO: 16538 - RNA, 3734 nt, Homo sapiens
  source 1..3734: mol_type = other RNA
gtgggcgggggcaggtgtgtggctgacagtggggagcctgctggggacgccaagggtgctgtttcctgcttaatcagggacacctctgtccccttctagctttccagggataactgggatgctcccacgccccctgtgtggctcagggatgaggcacttctctctcagccactcaactgatggaaggaaaaggcgatggaaagtctaacttttctgaaacaggtaggtgacaccttttggaaccggaatcaatcattattcttgcgtgggttttccattttccctgaagcatcgcaccagcttttgcgcgatgcctcggcttaccattttgcatctatcttaaggaattaggaggattcagaggagggtttctacgggcctctgctcacttttcacctctagggagactcaagtttccaagcattctttctgcaaagcacctgcctttgctaccttattgccgtattaccagccatcattttgattcatcttgaatactacagattaaaaaatattccctgcataatggctttgtgcaaaaacaagggaaagaaaacagaaagaagaaaggaaaatgtcctatcagaaagtggtcctccatgtttgcagaaaacccaggacccaccgggccctggtgggagcgggaagccgcctgccctgggagagggtgcccatcggtcaggatgcccggctggcctgcccagccccgctggcatagctacaggacgcccccgtggtaggcatggctgggggctgggctgccgaggctgtctgggcaggctttggtgttgtggtggttgcacggcggctcgtccttctgccgctccttctccatccaggtttccagcagctgctgcttgtcttgctcctcccgcatgaacagctccaccatgagcaccttctccttgtggatctgctggctgatgtccttggggatgtccgggatgacccagtccacaaagtcgctcatgaacatgaccaggttctggaagacgatgacaaacgccagccgggctgccaggacggcccagaagtccttggagatgtcgtacttgttttccgaccacggcggctctcggtagtctttatacctgcagatctgcacctcgtagcccaggtccagggggtcattgggggccgtgccgttctggaagtcactgacgttgaaggaggagagggtgtggttgacgaagccgtgcatggtcccgttcttactgtacatgtagaggtacaccaggcgcgggatgaagtcagacgtgaaggagatcacgaaggcattgatgatgacagcaagcttcccaatgcctctgaggatattgtaccagattccgatgtctttggctctgacagctaccggccttcggagctcagtgacaaactttttggcgtccaggcggatctcgatgatgttgttcagcagcgcaaacagtggggccagggggaaggaggcgacaaacagggtgacgaagccaaactggatgatcatttccatgtactctggggtgaggcccgcgaagggctccaggttgtaatccacctcgtaccgctgtttcctcttcacacactcctcgtggtcaggggggctctgctgcttcagcttcaggtagcggatgagcttcttcatcttcgggatgccgatctcgaacaggttgttctggatcagctgtttccccagcatgatgatgctgagctggatgcatagctccatcaggcagccccctggcgcacactcttccattcggaaggaacggaaaatgtacacgtagtcgcccgggcgtccaacaaaccggcctttgaagaacgccacgtaaaagatgggggtgtaggaattcacaaacttcagcaggaaagccttgaagatcagcctctcctcaaagcttttctccgtctttgggacctcgatcttggtgagccatcgggctatgcagccatacacctcgtccaggaggatgatgaccactaggttgatgatgactgcggtggctgtgactgtgacccggatgttggaccgcacggagggggaggagttcatggccaaggcggcggccatggagattctgtagatgatgacgccgaggacgatggcaaacgtcactgcaatcatgaagatgatggagaccaagttagtgaggtaggctgggaaccgatctctccatgtcagcttcactttgtcagtctctttgtttctggactctttcttcagagacttctccaagactctggcttcgtattcagctctaggatgatccttgacagcctcctcttcctcttcaaagcccgtgaggtcccagcggtagttgagtcgcatctgtttccgcttccagtgctccatgaaggtggcagcccagagggccatgaagacagagaagaagaccgtggcggggttgtcgaagaggtggctggcgcgggccgtggcgcaggctgagctcatcttccagtagctgcaggtcttgtcgcaaagcgggcacatggtgatattgtgtctctggtcacacatctccatgctggggatgttttcatccatggtggcgcatccgtacaggaagacaatgattcccacgatggaggcagggatgagcatctgggtgtacacgcccagccaggcgaagtacaggccgatcttctccccaaaatacttcctgaccaggtcgatgggctggtacttatagaaaactccatagcgtgcccactcttcgtacaggagttttctgtcgttgaactcgacgttttcaccgttgtagtctccatcgtgcagtgggtatgcagccgcgtacacaccattggccagcaggctcgtgatgccatacttcccacatttccgccttttacttagaagggcggagtccttctttcttccctcgccttgccccatgctgtacttggcctttgtacacgtcgttctcttcaagatctcatagacaatcgtgctccgggttttgctgtcgaaaaaggaatccttatcagacaagtcaaatagatgctgcttctcccgggagaagggataggagagtctcttcatggtctggggcctgtgctcagccactttgggctggatgggatctgtgattttctggagcacagagttgatttttttcaggaggccacgggtctcattaatgtggtacatcttcttcgtcggcatcttcagtttcagaaactcggcctctctgcacagcacgttccagggggcatggattttcacaaacccgactccgtggattttagtgtcctcgtcccgctccagctccaggcccgcctccaggaggttgccctcgtactcctccctgcggaagcgcttgtcatcctcgtggtagtccatcgggggctcccccgagcctgcatccagcgacgcccccttgcccggcagggggtggtcctgcttgacgctgcgagccccagagggggtgtcgctgtgctgcaccctcctgaccagggtccggttgcccgagggcctcttgtgatggtacaccaggatgtagtccaccttgcgccggccgtccctgaagtacaggccatacttgcactcggcatcagggtccacagataaggagttcagcagcgtgccctcggacggcaggtagccgatgtcctcgatggcgcagatgttgatgatgtggacgctgcggtcctcggccgggagcgtcgagtacttctcgttgaccctcatcgtggccgcctgtgcgctgggaccgccgggcggcgcgccctccccatccacggccccggcggcctct

SEQ ID NO: 16539 - RNA, 3614 nt, Homo sapiens
  source 1..3614: mol_type = other RNA
gtgggcgggggcaggtgtgtggctgacagtggggagcctgctggggacgccaagggtgctgtttcctgcttaatcagggacacctctgtccccttctagctttccagggataactgggatgctcccacgccccctgtgtggctcagggatgaggcacttctctctcagccactcaactgatggaaggaaaaggcgatggaaagtctaacttttctgaaacaggtaggtgacaccttttggaaccggaatcaatcattattcttgcgtgggttttccattttccctgaagcatcgcaccagcttttgcgcgatgcctcggcttaccattttgcatctatcttaaggaattaggaggattcagaggagggtttctacgggcctctgctcacttttcacctctagggagactcaagtttccaagcattctttctgcaaagcacctgcctttgctaccttattgccgtattaccagccatcattttgattcatcttgaatactacagattaaaaaatattccctgcataatggctttgtgcaaaaacaagggaaagaaaacagaaagaagaaaggaaaatgtcctatcagaaagtggtcctccatgtttgcagaaaacccaggacccaccgggccctggtgggagcgggaagccgcctgccctgggagagggtgcccatcggtcaggatgcccggctggcctgcccagccccgctggcatagctacaggacgcccccgtggtaggcatggctgggggctgggctgccgaggctgtctgggcaggctttggtgttgtggtggttgcacggcggctcgtccttctgccgctccttctccatccaggtttccagcagctgctgcttgtcttgctcctcccgcatgaacagctccaccatgagcaccttctccttgtggatctgctggctgatgtccttggggatgtccgggatgacccagtccacaaagtcgctcatgaacatgaccaggttctggaagacgatgacaaacgccagccgggctgccaggacggcccagaagtccttggagatgtcgtacttgttttccgaccacggcggctctcggtagtctttatacctgcagatctgcacctcgtagcccaggtccagggggtcattgggggccgtgccgttctggaagtcactgacgttgaaggaggagagggtgtggttgacgaagccgtgcatggtcccgttcttactgtacatgtagaggtacaccaggcgcgggatgaagtcagacgtgaaggagatcacgaaggcattgatgatgacagcaagcttcccaatgcctctgaggatattgtaccagattccgatgtctttggctctgacagctaccggccttcggagctcagtgacaaactttttggcgtccaggcggatctcgatgatgttgttcagcagcgcaaacagtggggccagggggaaggaggcgacaaacagggtgacgaagccaaactggatgatcatttccatgtactctggggtgaggcccgcgaagggctccaggttgtaatccacctcgtaccgctgtttcctcttcacacactcctcgtggtcaggggggctctgctgcttcagcttcaggtagcggatgagcttcttcatcttcgggatgccgatctcgaacaggttgttctggatcagctgtttccccagcatgatgatgctgagctggatgcatagctccatcaggcagccccctggcgcacactcttccattcggaaggaacggaaaatgtacacgtagtcgcccgggcgtccaacaaaccggcctttgaagaacgccacgtaaaagatgggggtgtaggaattcacaaacttcagcaggaaagccttgaagatcagcctctcctcaaagcttttctccgtctttgggacctcgatcttggtgagccatcgggctatgcagccatacacctcgtccaggaggatgatgaccactaggttgatgatgactgcggtggctgtgactgtgacccggatgttggaccgcacggagggggaggagttcatggccaaggcggcggccatggagattctgtagatgatgacgccgaggacgatggcaaacgtcactgcaatcatgaagatgatggagaccaagttagtgaggtaggctgggaaccgatctctccatgtcagcttcactttgtcagtctctttgtttctggactctttcttcagagacttctccaagactctggcttcgtattcagctctaggatgatccttgacagcctcctcttcctcttcaaagcccgtgaggtcccagcggtagttgagtcgcatctgtttccgcttccagtgctccatgaaggtggcagcccagagggccatgaagacagagaagaagaccgtggcggggttgtcgaagaggtggctggcgcgggccgtggcgcaggctgagctcatcttccagtagctgcaggtcttgtcgcaaagcgggcacatggtgatattgtgtctctggtcacacatctccatgctggggatgttttcatccatggtggcgcatccgtacaggaagacaatgattcccacgatggaggcagggatgagcatctgggtgtacacgcccagccaggcgaagtacaggccgatcttctccccaaaatacttcctgaccaggtcgatgggctggtacttatagaaaactccatagcgtgcccactcttcgtacaggagttttctgtcgttgaactcgacgttttcaccgttgtagtctccatcgtgcagtgggtatgcagccgcgtacacaccattggccagcaggctcgtgatgcccatgctgtacttggcctttgtacacgtcgttctcttcaagatctcatagacaatcgtgctccgggttttgctgtcgaaaaaggaatccttatcagacaagtcaaatagatgctgcttctcccgggagaagggataggagagtctcttcatggtctggggcctgtgctcagccactttgggctggatgggatctgtgattttctggagcacagagttgatttttttcaggaggccacgggtctcattaatgtggtacatcttcttcgtcggcatcttcagtttcagaaactcggcctctctgcacagcacgttccagggggcatggattttcacaaacccgactccgtggattttagtgtcctcgtcccgctccagctccaggcccgcctccaggaggttgccctcgtactcctccctgcggaagcgcttgtcatcctcgtggtagtccatcgggggctcccccgagcctgcatccagcgacgcccccttgcccggcagggggtggtcctgcttgacgctgcgagccccagagggggtgtcgctgtgctgcaccctcctgaccagggtccggttgcccgagggcctcttgtgatggtacaccaggatgtagtccaccttgcgccggccgtccctgaagtacaggccatacttgcactcggcatcagggtccacagataaggagttcagcagcgtgccctcggacggcaggtagccgatgtcctcgatggcgcagatgttgatgatgtggacgctgcggtcctcggccgggagcgtcgagtacttctcgttgaccctcatcgtggccgcctgt

SEQ ID NO: 16540 - RNA, 3569 nt, Homo sapiens
  source 1..3569: mol_type = other RNA
gtgggcgggggcaggtgtgtggctgacagtggggagcctgctggggacgccaagggtgctgtttcctgcttaatcagggacacctctgtccccttctagctttccagggataactgggatgctcccacgccccctgtgtggctcagggatgaggcacttctctctcagccactcaactgatggaaggaaaaggcgatggaaagtctaacttttctgaaacaggtaggtgacaccttttggaaccggaatcaatcattattcttgcgtgggttttccattttccctgaagcatcgcaccagcttttgcgcgatgcctcggcttaccattttgcatctatcttaaggaattaggaggattcagaggagggtttctacgggcctctgctcacttttcacctctagggagactcaagtttccaagcattctttctgcaaagcacctgcctttgctaccttattgccgtattaccagccatcattttgattcatcttgaatactacagattaaaaaatattccctgcataatggctttgtgcaaaaacaagggaaagaaaacagaaagaagaaaggaaaatgtcctatcagaaagtggtcctccatgtttgcagaaaacccaggacccaccgggccctggtgggagcgggaagccgcctgccctgggagagggtgcccatcggtcaggatgcccggctggcctgcccagccccgctggcatagctacaggacgcccccgtggtaggcatggctgggggctgggctgccgaggctgtctgggcaggctttggtgttgtggtggttgcacggcggctcgtccttctgccgctccttctccatccaggtttccagcagctgctgcttgtcttgctcctcccgcatgaacagctccaccatgagcaccttctccttgtggatctgctggctgatgtccttggggatgtccgggatgacccagtccacaaagtcgctcatgaacatgaccaggttctggaagacgatgacaaacgccagccgggctgccaggacggcccagaagtccttggagatgtcgtacttgttttccgaccacggcggctctcggtagtctttatacctgcagatctgcacctcgtagcccaggtccagggggtcattgggggccgtgccgttctggaagtcactgacgttgaaggaggagagggtgtggttgacgaagccgtgcatggtcccgttcttactgtacatgtagaggtacaccaggcgcgggatgaagtcagacgtgaaggagatcacgaaggcattgatgatgacagcaagcttcccaatgcctctgaggatattgtaccagattccgatgtctttggctctgacagctaccggccttcggagctcagtgacaaactttttggcgtccaggcggatctcgatgatgttgttcagcagcgcaaacagtggggccagggggaaggaggcgacaaacagggtgacgaagccaaactggatgatcatttccatgtactctggggtgaggcccgcgaagggctccaggttgtaatccacctcgtaccgctgtttcctcttcacacactcctcgtggtcaggggggctctgctgcttcagcttcaggtagcggatgagcttcttcatcttcgggatgccgatctcgaacaggttgttctggatcagctgtttccccagcatgatgatgctgagctggatgcatagctccatcaggcagccccctggcgcacactcttccattcggaaggaacggaaaatgtacacgtagtcgcccgggcgtccaacaaaccggcctttgaagaacgccacgtaaaagatgggggtgtaggaattcacaaacttcagcaggaaagccttgaagatcagcctctcctcaaagcttttctccgtctttgggacctcgatcttggtgagccatcgggctatgcagccatacacctcgtccaggaggatgatgaccactaggttgatgatgactgcggtggctgtgactgtgacccggatgttggaccgcacggagggggaggagttcatggccaaggcggcggccatggagattctgtagatgatgacgccgaggacgatggcaaacgtcactgcaatcatgaagatgatggagaccaagttagtgaggtaggctgggaaccgatctctccatgtcagcttcactttgtcagtctctttgtttctggactctttcttcagagacttctccaagactctggcttcgtattcagctctaggatgatccttgacagcctcctcttcctcttcaaagcccgtgaggtcccagcggtagttgagtcgcatctgtttccgcttccagtgctccatgaaggtggcagcccagagggccatgaagacagagaagaagaccgtggcggggttgtcgaagaggtggctggcgcgggccgtggcgcaggctgagctcatcttccagtagctgcaggtcttgtcgcaaagcgggcacatggtgatattgtgtctctggtcacacatctccatgctggggatgttttcatccatggtggcgcatccgtacaggaagacaatgattcccacgatggaggcagggatgagcatctgggtgtacacgcccagccaggcgaagtacaggccgatcttctccccaaaatacttcctgaccaggtcgatgggctggtacttatagaaaactccatagcgtgcccactcttcgtacaggagttttctgtcgttgaactcgacgttttcaccgttgtagtctccatcgtgcagtgggtatgcagccgcgtacacaccattggccagcaggctcgtgatgcccatgctgtacttggcctttgtacacgtcgttctcttcaagatctcatagacaatcgtgctccgggttttgctgtcgaaaaaggaatccttatcagacaagtcaaatagatgctgcttctcccgggagaagggataggagagtctcttcatggtctggggcctgtgctcagccactttgggctggatgggatctgtgattttctggagcacagagttgatttttttcaggaggccacgggtctcattaatgtggtacatgtcctcgtcccgctccagctccaggcccgcctccaggaggttgccctcgtactcctccctgcggaagcgcttgtcatcctcgtggtagtccatcgggggctcccccgagcctgcatccagcgacgcccccttgcccggcagggggtggtcctgcttgacgctgcgagccccagagggggtgtcgctgtgctgcaccctcctgaccagggtccggttgcccgagggcctcttgtgatggtacaccaggatgtagtccaccttgcgccggccgtccctgaagtacaggccatacttgcactcggcatcagggtccacagataaggagttcagcagcgtgccctcggacggcaggtagccgatgtcctcgatggcgcagatgttgatgatgtggacgctgcggtcctcggccgggagcgtcgagtacttctcgttgaccctcatcgtggccgcctgtgcgctgggaccgccgggcggcgcgccctccccatccacggccccggcggcctct

SEQ ID NO: 16541 - RNA, 5265 nt, Homo sapiens
  source 1..5265: mol_type = other RNA
gtgggctgggctgggctgggccagctgggagggccgaggagtctctgcactggcagttttgtaaacctgagcggggtagccaaccctcgagcccatgtcactgggctgcctcggtgggtctcggctgccccccgccagtcccgtgggggtgctggagccggaggagtacagcttcggtcggtagcccttgctttggccggcaactgcgggggcaggggagacctcccgccgcctgtctgcgtggtgggacctcccagcggcctcgcgacccccgccacaaaggcccatacttccagggggcttgtgtggcttggcgggccgtggagccttggccagggacatgcagctagggctggaggtgtagagggtggtgtcgatgccgctgtcactagagccacccttggagagggggtcttgctctggctccagggggtccagggggtcgaaccagcggtcgtcgctgtggctgctggatgcgttgctggagagggtgttgctgctggaatgacttgagtattgaggttctcctttggaatgcctgttgggggaatctttgcctgctgcatcctgcctggacgggtgcttgttcccgctgcttccggctatggctgagagcctggcctgggcaggcacatgccacaaaggctctggcttctggcgttccatggtgctctcctggctggtcaggccgccggaagaggagtcgccgctggacgtcccatcgtggctgaagtggggatcaagagatagcagggggtgtggggcagccgtgtacctttctggggatggcttgtatctcacgtaggtggccgaaccgggggtggagaagctcccagaaggctgtcggtagggagggactctgtcggcccctgctggtgatactgtgtaaggggtttctgggaagctgacaggcctcttgctgtgcagtggctgggactcccggaaggggactatgggggtctgcttcaggggccggctcagggactgggcatggccgggagtggttggagtggcccacttggaggctggtagagagttatgggatgcgggcccgctccactgccagggagcattgctgcggtaggggggccggcccccaggagtgatgctttcctgctccgtcttgggctccgaggtattcatgtcgtaggtctccggccaacccctccggggagtgccgtcctcaaaaggcgggatgatgaccaccttcacagtgacagaggtgcgcagcaggtcgatcatctggtcgtgggtcagtgtgaccacggccaccttgcagatctccactagtcggctgccctgccggaggccggcctgccaggcgaacccatagtcctcaacctcggccaccgtgccgtcgtacttcacgtggaagcccagctgcccgagcccgttccgccgaagcgtcatgtccaccgtctcccagccactggtcatcaccttcagtctctgcactatctcccttatgtcctccacagaaccctctgtcgcctgtaggaagatgtggtctcctcgtccatagaagattttgagtgtggaggagtctggagtccagccaatgacatccccgcagtagcagttgaacaccacctccttggtgcgtaagtccaggagcaccacaaactcattggaaattcccaaaatgcagtcgatttccaccccctgggcgtagtcctgggccaccaccctccaggcgatggcccctgcactgtgctgctcagcgccagcccgtgcttttgtcttttccttcttcttggaggtcagggagatgaggttgaatttgccggtggagtcgatgggggtgttggagacacagttttcggccaggtccttgagatactcctggcgggtcctggtggccatggtgtggaacttgtcggacttgtgcgcggcgttctcagcgttaatcaccttggccagcaagaagtctctgaagacgtcggatttgcggaatgtggttccactggggatgggggggccgaaaggaggagcgtctttggatcgggtcacagccatactgtaacagacgttatcagtgcaggggttgtggactcggacaatgatgaagacgtgctggaagtgggagcggatgttcttgggggtgaacggtagcgcgccaggctcctggaagatgatcgtcacgatgtcatttcctatgtgcctcttccgtagcagctgctgcctgttgttgggggtgtaagggagcagggtggagacatggaacatgatctcgtagtcctggtacatcgtgtagagggagtgggttcccgtggagtcggtcttgacgtccagctgggcagcgtacttggtgaagcccttcaggcagaccttctcgccgatgagggagaggaactcctcaaaggcggggccggcctcctcattgttgtacatctcctcctcggagctctggccggccttgcaatagaggatgcccaccttgtgcttccggcagagcccttgctcatcgagcttcagcagttgctccgtcaccttgggggtgttgagggccagccgcaggcagtggatgttgagctcggggatgacatactccagggcatccttcaagggcaggccccgcccggtcccatgcttggtggctgtgggcgtagcatcttccaggatggagccccgcagggtgatgagctcgcgggtccggaagatgatcctgtactggtactgaggtccgtgctccttgtggtcttccagcttctcccgcttaatgctcacagccactggccccagcttctcatccacgccgaagtaattggcatgttctttgcccacgaagtaatcctggtagtagcgggcgcccaggtccacatgctcgatgctgtactgccggggccgactctgcgtccgctgctgctccttgggaacttccaacaccgagatgctggcgttggtgcggtaggcgctcagggcgggctctgccaggtggccctcgccgctgctcggggagcccacggaagcccgggagaagctcacgttgcgctcacactcgcccccgatctcattgcggaagtgcgggcagctgagcagcaggtcgttgctgttgtcatcgccgaggtcctgctccaagttctccttgcagtttaggtcctctgtgctggtgaaggccgggtccaggcctccgaggctgtgggcccgcgaggccgtgagggaggccatggccgaggcggcggaagcggccgaagcacccgtggtggtgttccgccgctgcgacaccgacaccctgttggcggccgcctcgttgaggtcgaacagcatgctctgcacgtcgaagtgggcgaagctcttctgacacacccacggcctgctggcttccggggggctccggccctcgtcggcctcccccggggaacgcccagcctccccctcgggtttgctgctccttagcttccgaaagatggacgagtccaccgtgtccccgccgccgaggccccgcgcaggtttcttccgggccttctccttctccttcgtgggctgcagtggcaggaggctgtccttggcgggctgcccgttgtgggagtcccccttggctccgccgccgccccccatgaggtgtgggccaggatctgcccggaggagctcggtgagggcctggcaccctcgggcgtcgggctgctcgctgcggaactcgttcaggatgtcgaagaagctctgctcgggcatgccctgcacgtcgatggacgaggtgctcccgtactcgcggaagaggggcagcgcccccgtgtgccgggccccccgcggctcccccgcgtcctccgcgtcacactcgctgagggtgatctcgctgctgctgcggtgccgaagggggaggaaggccctgccgggggaccggggccacccgtcctggaactccacgtctttggaccttctcctggagagtcggtggaaggctttggaccctgaggaagccggggtgctggtggggggctgtccgttctgtatgctcctcatggaatgggccatcttggtggcctttgtgccatctgtgtcctgggaggggcttgggttgctgtgctctctcagggcctcccgcttgggcggccagtcggccacccttgcgcgcacgcccatcttgggcattgcgggagtggtggggctggggcgggtggtggcggtggcggtggcggtggcggtggccgggctctcgccaagaggctgggacatgctgccattctgggcccagaatcccaagggagcgtagtcccctgtgtgtggcccagggaggacatcgcccaccctggcgccacagctggctgccaggtccacaccatcgctggggatggcccgataggtggtcatagtccacgggcactggagtgctgctggccccgtacgctgtggtgtcactctatggggtcccccagccctcagccattgttcagggcagccaggcccaggatgaaggatgctgggccctgaaacctgacaggaaggttgtgagcctgtggagtccagttctccaccatcgctgtgcacagctgagccaggacaacctcaggaagcaggtgctgtcctgggggctccagaccgagtggctcagtagcgcagagcaggcagtagctgtggtcgcccgccagctggaggcagcaaggatgttgtcctcgccatgccttagtgccttctagacactagtgctcttggagggtcccaggagagctgatgtcagagactgtgcatctcttccccagtcagaacaccagtgggctttgcagtttgttcttcatttcttagagtccatgaaaagagggcaaggcctctgggggcctgaggtccgcatctgcaataggaggataacattcagtcttcagacgcactcacattcattcaacatgcactcatgaagcaactgctatgggccaggcactgctctagacgctggggatacagaaaggaacaaagacaaagatccctgccttcacggagctcacattccaaggaggatggtgtagaaagcaaatatagaacatcagaccgtgataaacaccatgaagaaaaataaagcagaagacagcgacagggagggccattttagacagggtgctgaggaaggccgctcagagatggtgtctcagagatctcaataaagtaactaaatcatacatgcacacacatgcacacacacaccaagatacttacacacatgtagccaagaacacagtgcctggtatggaaaatgaaggtgatctaatttgacagttaagagtgctctaacagggtatgcttaagttaagcaaaaaaaggtagaagaagaattaa

SEQ ID NO: 16542 - RNA, 5619 nt, Homo sapiens
  source 1..5619: mol_type = other RNA
gtgggctgggctgggctgggccagctgggagggccgaggagtctctgcactggcagttttgtaaacctgagcggggtagccaaccctcgagcccatgtcactgggctgcctcggtgggtctcggctgccccccgccagtcccgtgggggtgctggagccggaggagtacagcttcggtcggtagcccttgctttggccggcaactgcgggggcaggggagacctcccgccgcctgtctgcgtggtgggacctcccagcggcctcgcgacccccgccacaaaggcccatacttccagggggcttgtgtggcttggcgggccgtggagccttggccagggacatgcagctagggctggaggtgtagagggtggtgtcgatgccgctgtcactagagccacccttggagagggggtcttgctctggctccagggggtccagggggtcgaaccagcggtcgtcgctgtggctgctggatgcgttgctggagagggtgttgctgctggaatgacttgagtattgaggttctcctttggaatgcctgttgggggaatctttgcctgctgcatcctgcctggacgggtgcttgttcccgctgcttccggctatggctgagagcctggcctgggcaggcacatgccacaaaggctctggcttctggcgttccatggtgctctcctggctggtcaggccgccggaagaggagtcgccgctggacgtcccatcgtggctgaagtggggatcaagagatagcagggggtgtggggcagccgtgtacctttctggggatggcttgtatctcacgtaggtggccgaaccgggggtggagaagctcccagaaggctgtcggtagggagggactctgtcggcccctgctggtgatactgtgtaaggggtttctgggaagctgacaggcctcttgctgtgcagtggctgggactcccggaaggggactatgggggtctgcttcaggggccggctcagggactgggcatggccgggagtggttggagtggcccacttggaggctggtagagagttatgggatgcgggcccgctccactgccagggagcattgctgcggtaggggggccggcccccaggagtgatgctttcctgctccgtcttgggctccgaggtattcatgtcgtaggtctccggccaacccctccggggagtgccgtcctcaaaaggcgggatgatgaccaccttcacagtgacagaggtgcgcagcaggtcgatcatctggtcgtgggtcagtgtgaccacggccaccttgcagatctccactagtcggctgccctgccggaggccggcctgccaggcgaacccatagtcctcaacctcggccaccgtgccgtcgtacttcacgtggaagcccagctgcccgagcccgttccgccgaagcgtcatgtccaccgtctcccagccactggtcatcaccttcagtctctgcactatctcccttatgtcctccacagaaccctctgtcgcctgtaggaagatgtggtctcctcgtccatagaagattttgagtgtggaggagtctggagtccagccaatgacatccccgcagtagcagttgaacaccacctccttggtgcgtaagtccaggagcaccacaaactcattggaaattcccaaaatgcagtcgatttccaccccctgggcgtagtcctgggccaccaccctccaggcgatggcccctgcactgtgctgctcagcgccagcccgtgcttttgtcttttccttcttcttggaggtcagggagatgaggttgaatttgccggtggagtcgatgggggtgttggagacacagttttcggccaggtccttgagatactcctggcgggtcctggtggccatggtgtggaacttgtcggacttgtgcgcggcgttctcagcgttaatcaccttggccagcaagaagtctctgaagacgtcggatttgcggaatgtggttccactggggatgggggggccgaaaggaggagcgtctttggatcgggtcacagccatactgtaacagacgttatcagtgcaggggttgtggactcggacaatgatgaagacgtgctggaagtgggagcggatgttcttgggggtgaacggtagcgcgccaggctcctggaagatgatcgtcacgatgtcatttcctatgtgcctcttccgtagcagctgctgcctgttgttgggggtgtaagggagcagggtggagacatggaacatgatctcgtagtcctggtacatcgtgtagagggagtgggttcccgtggagtcggtcttgacgtccagctgggcagcgtacttggtgaagcccttcaggcagaccttctcgccgatgagggagaggaactcctcaaaggcggggccggcctcctcattgttgtacatctcctcctcggagctctggccggccttgcaatagaggatgcccaccttgtgcttccggcagagcccttgctcatcgagcttcagcagttgctccgtcaccttgggggtgttgagggccagccgcaggcagtggatgttgagctcggggatgacatactccagggcatccttcaagggcaggccccgcccggtcccatgcttggtggctgtgggcgtagcatcttccaggatggagccccgcagggtgatgagctcgcgggtccggaagatgatcctgtactggtactgaggtccgtgctccttgtggtcttccagcttctcccgcttaatgctcacagccactggccccagcttctcatccacgccgaagtaattggcatgttctttgcccacgaagtaatcctggtagtagcgggcgcccaggtccacatgctcgatgctgtactgccggggccgactctgcgtccgctgctgctccttgggaacttccaacaccgagatgctggcgttggtgcggtaggcgctcagggcgggctctgccaggtggccctcgccgctgctcggggagcccacggaagcccgggagaagctcacgttgcgctcacactcgcccccgatctcattgcggaagtgcgggcagctgagcagcaggtcgttgctgttgtcatcgccgaggtcctgctccaagttctccttgcagtttaggtcctctgtgctggtgaaggccgggtccaggcctccgaggctgtgggcccgcgaggccgtgagggaggccatggccgaggcggcggaagcggccgaagcacccgtggtggtgttccgccgctgcgacaccgacaccctgttggcggccgcctcgttgaggtcgaacagcatgctctgcacgtcgaagtgggcgaagctcttctgacacacccacggcctgctggcttccggggggctccggccctcgtcggcctcccccggggaacgcccagcctccccctcgggtttgctgctccttagcttccgaaagatggacgagtccaccgtgtccccgccgccgaggccccgcgcaggtttcttccgggccttctccttctccttcgtgggctgcagtggcaggaggctgtccttggcgggctgcccgttgtgggagtcccccttggctccgccgccgccccccatgaggtgtgggccaggatctgcccggaggagctcggtgagggcctggcaccctcgggcgtcgggctgctcgctgcggaactcgttcaggatgtcgaagaagctctgctcgggcatgccctgcacgtcgatggacgaggtgctcccgtactcgcggaagaggggcagcgcccccgtgtgccgggccccccgcggctcccccgcgtcctccgcgtcacactcgctgagggtgatctcgctgctgctgcggtgccgaagggggaggaaggccctgccgggggaccggggccacccgtcctggaactccacgtctttggaccttctcctggagagtcggtggaaggctttggaccctgaggaagccggggtgctggtggggggctgtccgttctgtatgctcctcatggaatgggccatcttggtggcctttgtgccatctgtgtcctgggaggggcttgggttgctgtgctctctcagggcctcccgcttgggcggccagtcggccacccttgcgcgcacgcccatcttgggcattgcgggagtggtggggctggggcgggtggtggcggtggcggtggcggtggcggtggccgggctctcgccaagaggctgggacatgctgccattctgggcccagaatcccaagggagcgtagtcccctgtgtgtggcccagggaggacatcgcccaccctggcgccacagctggctgccaggtccacaccatcgctggggatggcccgataggtggtcatagtccacgggcactggagtgctgctggccccgtacgctgtggtgtcactctatggggtcccccagccctcagccattgttcagggcagccaggcccaggatgaaggatgctgggccctgaaacctgacaggaaggttgtgagcctgtggagtccagttctccaccatcgctgtgcacagctgagccaggacaacctcaggaagcaggtgctgtcctgggggctccagaccgagtggctcagtagcgcagagcaggcagtagctgtggtcgcccgccagctggaggcagcaaggatgttgtcctcgccatgccttagtgccttctagacactagtgctcttggagggtcccaggagagctgatgtcagagactgtgcatctgaaagactccccgaacacggctctgatcacaaagtgggcaggtggctgtcaggggagccccaggtggactcctcctgtccctggtcctcccagggcgaggccacctgccttggctctccaggccgacctcagtggtgcccgcccccagcccgctgtgggtgcctggaatgcggaaacgggaacctgccgtgccagctcctaacagcgacttattcaacagccgcaggaacacgccagccagccaccggagttccccaggagatggctggtcgtcgtgaacaggcgcgttcccaaagaaagctgttttgccaacattccctttgggggagggaaagaaaaggcctccttactcatcagacacgtggtctgaggagtctgaatgggcttgaaagaaagctcaaaggtaacaaaggcggctcgcctattacctcggattcaggcacaggccacctgttcactgacagagccagggctggacttgtgcccacaccgtcccctgccctgagcttgcgcctggatgcttcattcagaaccgtacaatctaaaggcgggctccttggcccgtgcagaggaggcactagctcacagaggcaatgcagcttaatgattaaacacggtcgctggactcttccagccagctttggaagcacaactgaacggctttggctggctaataataacaaccacaaccggaatgctcactgcacaaggcgctgttctaagtgctacatatgaattctctctcctaaccctcacagcgaccctctaaggaggaactatcagcattcttattttacagatgagaagttcaacgaataagtcataggctggaggtcacacaggaagaaagtgctggggtggggatctaacccaagcagaggagctccaaggttccagtttttacccactactttatttatttattttattt

SEQ ID NO: 16543 - RNA, 4837 nt, Homo sapiens
  source 1..4837: mol_type = other RNA
gtgggctgggctgggctgggccagctgggagggccgaggagtctctgcactggcagttttgtaaacctgagcggggtagccaaccctcgagcccatgtcactgggctgcctcggtgggtctcggctgccccccgccagtcccgtgggggtgctggagccggaggagtacagcttcggtcggtagcccttgctttggccggcaactgcgggggcaggggagacctcccgccgcctgtctgcgtggtgggacctcccagcggcctcgcgacccccgccacaaaggcccatacttccagggggcttgtgtggcttggcgggccgtggagccttggccagggacatgcagctagggctggaggtgtagagggtggtgtcgatgccgctgtcactagagccacccttggagagggggtcttgctctggctccagggggtccagggggtcgaaccagcggtcgtcgctgtggctgctggatgcgttgctggagagggtgttgctgctggaatgacttgagtattgaggttctcctttggaatgcctgttgggggaatctttgcctgctgcatcctgcctggacgggtgcttgttcccgctgcttccggctatggctgagagcctggcctgggcaggcacatgccacaaaggctctggcttctggcgttccatggtgctctcctggctggtcaggccgccggaagaggagtcgccgctggacgtcccatcgtggctgaagtggggatcaagagatagcagggggtgtggggcagccgtgtacctttctggggatggcttgtatctcacgtaggtggccgaaccgggggtggagaagctcccagaaggctgtcggtagggagggactctgtcggcccctgctggtgatactgtgtaaggggtttctgggaagctgacaggcctcttgctgtgcagtggctgggactcccggaaggggactatgggggtctgcttcaggggccggctcagggactgggcatggccgggagtggttggagtggcccacttggaggctggtagagagttatgggatgcgggcccgctccactgccagggagcattgctgcggtaggggggccggcccccaggagtgatgctttcctgctccgtcttgggctccgaggtattcatgtcgtaggtctccggccaacccctccggggagtgccgtcctcaaaaggcgggatgatgaccaccttcacagtgacagaggtgcgcagcaggtcgatcatctggtcgtgggtcagtgtgaccacggccaccttgcagatctccactagtcggctgccctgccggaggccggcctgccaggcgaacccatagtcctcaacctcggccaccgtgccgtcgtacttcacgtggaagcccagctgcccgagcccgttccgccgaagcgtcatgtccaccgtctcccagccactggtcatcaccttcagtctctgcactatctcccttatgtcctccacagaaccctctgtcgcctgtaggaagatgtggtctcctcgtccatagaagattttgagtgtggaggagtctggagtccagccaatgacatccccgcagtagcagttgaacaccacctccttggtgcgtaagtccaggagcaccacaaactcattggaaattcccaaaatgcagtcgatttccaccccctgggcgtagtcctgggccaccaccctccaggcgatggcccctgcactgtgctgctcagcgccagcccgtgcttttgtcttttccttcttcttggaggtcagggagatgaggttgaatttgccggtggagtcgatgggggtgttggagacacagttttcggccaggtccttgagatactcctggcgggtcctggtggccatggtgtggaacttgtcggacttgtgcgcggcgttctcagcgttaatcaccttggccagcaagaagtctctgaagacgtcggatttgcggaatgtggttccactggggatgggggggccgaaaggaggagcgtctttggatcgggtcacagccatactgtaacagacgttatcagtgcaggggttgtggactcggacaatgatgaagacgtgctggaagtgggagcggatgttcttgggggtgaacggtagcgcgccaggctcctggaagatgatcgtcacgatgtcatttcctatgtgcctcttccgtagcagctgctgcctgttgttgggggtgtaagggagcagggtggagacatggaacatgatctcgtagtcctggtacatcgtgtagagggagtgggttcccgtggagtcggtcttgacgtccagctgggcagcgtacttggtgaagcccttcaggcagaccttctcgccgatgagggagaggaactcctcaaaggcggggccggcctcctcattgttgtacatctcctcctcggagctctggccggccttgcaatagaggatgcccaccttgtgcttccggcagagcccttgctcatcgagcttcagcagttgctccgtcaccttgggggtgttgagggccagccgcaggcagtggatgttgagctcggggatgacatactccagggcatccttcaagggcaggccccgcccggtcccatgcttggtggctgtgggcgtagcatcttccaggatggagccccgcagggtgatgagctcgcgggtccggaagatgatcctgtactggtactgaggtccgtgctccttgtggtcttccagcttctcccgcttaatgctcacagccactggccccagcttctcatccacgccgaagtaattggcatgttctttgcccacgaagtaatcctggtagtagcgggcgcccaggtccacatgctcgatgctgtactgccggggccgactctgcgtccgctgctgctccttgggaacttccaacaccgagatgctggcgttggtgcggtaggcgctcagggcgggctctgccaggtggccctcgccgctgctcggggagcccacggaagcccgggagaagctcacgttgcgctcacactcgcccccgatctcattgcggaagtgcgggcagctgagcagcaggtcgttgctgttgtcatcgccgaggtcctgctccaagttctccttgcagtttaggtcctctgtgctggtgaaggccgggtccaggcctccgaggctgtgggcccgcgaggccgtgagggaggccatggccgaggcggcggaagcggccgaagcacccgtggtggtgttccgccgctgcgacaccgacaccctgttggcggccgcctcgttgaggtcgaacagcatgctctgcacgtcgaagtgggcgaagctcttctgacacacccacggcctgctggcttccggggggctccggccctcgtcggcctcccccggggaacgcccagcctccccctcgggtttgctgctccttagcttccgaaagatggacgagtccaccgtgtccccgccgccgaggccccgcgcaggtttcttccgggccttctccttctccttcgtgggctgcagtggcaggaggctgtccttggcgggctgcccgttgtgggagtcccccttggctccgccgccgccccccatgaggtgtgggccaggatctgcccggaggagctcggtgagggcctggcaccctcgggcgtcgggctgctcgctgcggaactcgttcaggatgtcgaagaagctctgctcgggcatgccctgcacgtcgatggacgaggtgctcccgtactcgcggaagaggggcagcgcccccgtgtgccgggccccccgcggctcccccgcgtcctccgcgtcacactcgctgagggtgatctcgctgctgctgcggtgccgaagggggaggaaggccctgccgggggaccggggccacccgtcctggaactccacgtctttggaccttctcctggagagtcggtggaaggctttggaccctgaggaagccggggtgctggtggggggctgtccgttctgtatgctcctcatggaatgggccatcttggtggcctttgtgccatctgtgtcctgggaggggcttgggttgctgtgctctctcagggcctcccgcttgggcggccagtcggccacccttgcgcgcacgcccatcttgggcattgcgggagtggtggggctggggcgggtggtggcggtggcggtggcggtggcggtggccgggctctcgccaagaggctgggacatgctgccattctgggcccagaatcccaagggagcgtagtcccctgtgtgtggcccagggaggacatcgcccaccctggcgccacagctggctgccaggtccacaccatcgctggggatggcccgataggtggtcatagtccacgggcactggagtgctgctggccccgtacgctgtggtgtcactctatggggtcccccagccctcagccattgttcagggcagccaggcccaggatgaaggatgctgggccctgaaacctgacaggaaggttgtgagcctgtggagtccagttctccaccatcgctgtgcacagctgagccaggacaacctcaggaagcaggtgctgtcctgggggctccagaccgagtggctcagtagcgcagagcaggcagtagctgtggtcgcccgccagctggaggcagcaaggatgttgtcctcgccatgccttagtgccttctagacactagtgctcttggagggtcccaggagagctgatgtcagagactgtgcatctggacgccccggctgcccgcctcgcgggccccacgatcgcggcgtccagctccgcgccgctcgctggagacgccgccagctccggtggcccgagtgacttccaggctgcccacttccaagccgcttcgcgcgagtcctcctgggaactgt

SEQ ID NO: 16544 - RNA, 5222 nt, Homo sapiens
  source 1..5222: mol_type = other RNA
gtgggctgggctgggctgggccagctgggagggccgaggagtctctgcactggcagttttgtaaacctgagcggggtagccaaccctcgagcccatgtcactgggctgcctcggtgggtctcggctgccccccgccagtcccgtgggggtgctggagccggaggagtacagcttcggtcggtagcccttgctttggccggcaactgcgggggcaggggagacctcccgccgcctgtctgcgtggtgggacctcccagcggcctcgcgacccccgccacaaaggcccatacttccagggggcttgtgtggcttggcgggccgtggagccttggccagggacatgcagctagggctggaggtgtagagggtggtgtcgatgccgctgtcactagagccacccttggagagggggtcttgctctggctccagggggtccagggggtcgaaccagcggtcgtcgctgtggctgctggatgcgttgctggagagggtgttgctgctggaatgacttgagtattgaggttctcctttggaatgcctgttgggggaatctttgcctgctgcatcctgcctggacgggtgcttgttcccgctgcttccggctatggctgagagcctggcctgggcaggcacatgccacaaaggctctggcttctggcgttccatggtgctctcctggctggtcaggccgccggaagaggagtcgccgctggacgtcccatcgtggctgaagtggggatcaagagatagcagggggtgtggggcagccgtgtacctttctggggatggcttgtatctcacgtaggtggccgaaccgggggtggagaagctcccagaaggctgtcggtagggagggactctgtcggcccctgctggtgatactgtgtaaggggtttctgggaagctgacaggcctcttgctgtgcagtggctgggactcccggaaggggactatgggggtctgcttcaggggccggctcagggactgggcatggccgggagtggttggagtggcccacttggaggctggtagagagttatgggatgcgggcccgctccactgccagggagcattgctgcggtaggggggccggcccccaggagtgatgctttcctgctccgtcttgggctccgaggtattcatgtcgtaggtctccggccaacccctccggggagtgccgtcctcaaaaggcgggatgatgaccaccttcacagtgacagaggtgcgcagcaggtcgatcatctggtcgtgggtcagtgtgaccacggccaccttgcagatctccactagtcggctgccctgccggaggccggcctgccaggcgaacccatagtcctcaacctcggccaccgtgccgtcgtacttcacgtggaagcccagctgcccgagcccgttccgccgaagcgtcatgtccaccgtctcccagccactggtcatcaccttcagtctctgcactatctcccttatgtcctccacagaaccctctgtcgcctgtaggaagatgtggtctcctcgtccatagaagattttgagtgtggaggagtctggagtccagccaatgacatccccgcagtagcagttgaacaccacctccttggtgcgtaagtccaggagcaccacaaactcattggaaattcccaaaatgcagtcgatttccaccccctgggcgtagtcctgggccaccaccctccaggcgatggcccctgcactgtgctgctcagcgccagcccgtgcttttgtcttttccttcttcttggaggtcagggagatgaggttgaatttgccggtggagtcgatgggggtgttggagacacagttttcggccaggtccttgagatactcctggcgggtcctggtggccatggtgtggaacttgtcggacttgtgcgcggcgttctcagcgttaatcaccttggccagcaagaagtctctgaagacgtcggatttgcggaatgtggttccactggggatgggggggccgaaaggaggagcgtctttggatcgggtcacagccatactgtaacagacgttatcagtgcaggggttgtggactcggacaatgatgaagacgtgctggaagtgggagcggatgttcttgggggtgaacggtagcgcgccaggctcctggaagatgatcgtcacgatgtcatttcctatgtgcctcttccgtagcagctgctgcctgttgttgggggtgtaagggagcagggtggagacatggaacatgatctcgtagtcctggtacatcgtgtagagggagtgggttcccgtggagtcggtcttgacgtccagctgggcagcgtacttggtgaagcccttcaggcagaccttctcgccgatgagggagaggaactcctcaaaggcggggccggcctcctcattgttgtacatctcctcctcggagctctggccggccttgcaatagaggatgcccaccttgtgcttccggcagagcccttgctcatcgagcttcagcagttgctccgtcaccttgggggtgttgagggccagccgcaggcagtggatgttgagctcggggatgacatactccagggcatccttcaagggcaggccccgcccggtcccatgcttggtggctgtgggcgtagcatcttccaggatggagccccgcagggtgatgagctcgcgggtccggaagatgatcctgtactggtactgaggtccgtgctccttgtggtcttccagcttctcccgcttaatgctcacagccactggccccagcttctcatccacgccgaagtaattggcatgttctttgcccacgaagtaatcctggtagtagcgggcgcccaggtccacatgctcgatgctgtactgccggggccgactctgcgtccgctgctgctccttgggaacttccaacaccgagatgctggcgttggtgcggtaggcgctcagggcgggctctgccaggtggccctcgccgctgctcggggagcccacggaagcccgggagaagctcacgttgcgctcacactcgcccccgatctcattgcggaagtgcgggcagctgagcagcaggtcgttgctgttgtcatcgccgaggtcctgctccaagttctccttgcagtttaggtcctctgtgctggtgaaggccgggtccaggcctccgaggctgtgggcccgcgaggccgtgagggaggccatggccgaggcggcggaagcggccgaagcacccgtggtggtgttccgccgctgcgacaccgacaccctgttggcggccgcctcgttgaggtcgaacagcatgctctgcacgtcgaagtgggcgaagctcttctgacacacccacggcctgctggcttccggggggctccggccctcgtcggcctcccccggggaacgcccagcctccccctcgggtttgctgctccttagcttccgaaagatggacgagtccaccgtgtccccgccgccgaggccccgcgcaggtttcttccgggccttctccttctccttcgtgggctgcagtggcaggaggctgtccttggcgggctgcccgttgtgggagtcccccttggctccgccgccgccccccatgaggtgtgggccaggatctgcccggaggagctcggtgagggcctggcaccctcgggcgtcgggctgctcgctgcggaactcgttcaggatgtcgaagaagctctgctcgggcatgccctgcacgtcgatggacgaggtgctcccgtactcgcggaagaggggcagcgcccccgtgtgccgggccccccgcggctcccccgcgtcctccgcgtcacactcgctgagggtgatctcgctgctgctgcggtgccgaagggggaggaaggccctgccgggggaccggggccacccgtcctggaactccacgtctttggaccttctcctggagagtcggtggaaggctttggaccctgaggaagccggggtgctggtggggggctgtccgttctgtatgctcctcatggaatgggccatcttggtggcctttgtgccatctgtgtcctgggaggggcttgggttgctgtgctctctcagggcctcccgcttgggcggccagtcggccacccttgcgcgcacgcccatcttgggcattgcgggagtggtggggctggggcgggtggtggcggtggcggtggcggtggcggtggccgggctctcgccaagaggctgggacatgctgccattctgggcccagaatcccaagggagcgtagtcccctgtgtgtggcccagggaggacatcgcccaccctggcgccacagctggctgccaggtccacaccatcgctggggatggcccgataggtggtcatagtccacgggcactggagtgctgctggccccgtacgctgtggtgtcactctatggggtcccccagccctcagccattgttcagggcagccaggcccaggatgaaggatgctgggccctgaaacctgacaggaaggttgtgagcctgtggagtccagttctccaccatcgctgtgcacagctgagccaggacaacctcaggaagcaggtgctgtcctgggggctccagaccgagtggctcagtagcgcagagcaggcagtagctgtggtcgcccgccagctggaggcagcaaggatgttgtcctcgccatgccttagtgccttctagacactagtgctcttggagggtcccaggagagctgatgtcagagactgtgcatctggacgccccggctgcccgcctcgcgggccccacgatcgcggcgtccagctccgcgccgctcgctggagacgccgccagctccggtggcccgagtgacttccaggctgcccacttccaagccgcttcgcgcgagtcctcctgggaactgtagtttcgccctagccggccgcgaactcaaaaagagaatggcgcgcgggggctgccgggagccgtaggcgcaccgccgcgctgcctcctaggaacggtagtccgctggtcgccttcgtgcagctccagtctgtagagcacttccgcagccccgaggggcgtgagggagggaggtgtgtctcctgcagactacagctcgagagccgcgctcttcgccccgccggggcggtttctcctttctcctggccccgtctacctcctcccttcattcggcggaacctctccctcactctctgccaggctcgagtcacttacccctaggacgctagcccgggggaaacgggggaagcggagcagtgcgctagacccccagcggagggggcggtg

SEQ ID NO: 16545 - RNA, 3371 nt, Homo sapiens
  source 1..3371: mol_type = other RNA
gtgggctgggctgggctgggccaggcctggggccacagtctcttcctgcttctggtttgcagagaaagaagaaagcaaggagatggaggagcaggcagttaccccgcagaaagaggaactagagacagtggccccaccagagccagagccaagtgaggatctggagagggcaggctgccctgtccctctgagcaggtgtagaatgaagggtttggatgacatcaggacttcagactttttgtttttagtcagagtcctttctctaaatgatcccttatgcagaagtccaagatgacagataaaagcacagctgcaggccaggcgtggtggctcacacctgtaatcccagcacaatctgaggcaggcggattgcctgagctcaggagttcgcgaccagcctgggcaacaccgtgaaaccccctatctactaaaatacaaaaaatagccaggcatggtggtgcgcgcttgtagtcccagctactcaggaggctgaggcaggagaactgcatgaacccaggaggtggagactgcagtgagccaagatctggccactgcactccagcctgggcaacagagcaagactctgtctcaaaacaaacaaacaaacaaacaaaaagcacagctgaagtggctccagagaaatgatcattagaaagccaatgacggtggcttaaaacctatatgatgggttgatgggtaaagcaaaccaccatggcccatgtatacctacgtagcaaacctgcatgttctgctcgtatcccagaacttaagagttaaaaaaaaacaaagaacaggccaggtgcagtggctcacaactgtaatcccagcactttgggaggctgaggcaggcggatcacgaggtcaggagatcgagtccatcctggctaacactgtgaaaccccgtctctactaaaaatacaaaaagttagccgggcgtggtggcgggtgcctgtagtcccagctactgggaggctgaggcaggagaatggcatgaacctgggaggcagagcttgcagtgagctgagatcgctgccactgcactccagcctgggggataaagcaagactccatctcaaaaaaaaaaaaaaaaagagaaagccaatgacaataacagccagcacatacttggcaataggtgtgcagtgcatgccctgctctaagcattttacataaattaactcatttaatcctccctcaatcctatgtgctaggtatcactatccacatttcatacaaggaaactgaggcacagataggttaaataacctgcctaaggtcacacagctactgagtagggatcagaatttgaagctgcaaagtccagcatagccaccctacccaactacctctcacacaagggcttgctaacatttcctaaagggaaacaacattgctacctctatatccccaccaggggaaatttggggactgtttgcccaactagggaccatccccccattgccagacagcatctctcctcaccctgccccttcttccctgcccctgcaggccacatccacgtcctccgagcctacatcaagacccaagtgaacaaagagctggagcagctccaggggctggtggaggagcggctcaaggccagcgaggaaaggctcagcagcaagttgactgcactagagcggcccttccagctacctccgggtaaaggcaagagcaagaccaagtgacccccaacattttccccaataaaggtctgggccagaatggcaccatccctgcaccctgctgagcaccttctgggctttcctgcccaagccagacagacacaggacacctgttctccctggcgtgtagcagattttatttcatatgcagtgcatgcagcactgaccgggccaggcgtggcgttcagaatggctcccttccaccccagctctgatctcagagtcctggccagtggggagagaggtaccgggctggtcttcaagagggtagcaggatcattagtgggcctgaggccagaggccagagcccagaggagctggaatgatcaaaacccttcttctggagagttctgcttcctgggaatccctggggttgaggtcctagcccagcacaagcacggcctcatcctcagttatagcagcagagtctccctcctcttcagggcccatgatgggaaaaggcccagggggccggtgctgaaagagagccgcccggttctgctgctcccctttctttacccagtgcccgtagagccggaaggcacagttgtcgatgaggtgccgcactgaccgcagcgcataagggtccctcaacagtgcattcttggtcagtggccgtacacgatgggtgcttagggccactcgtccagcagccagcactgtccacactgccacccggaaccgctggcggggggtgaggttccagggttggctgccttcacaacgctcaaagaaggggtgctgtagggcctgctcagctgtcaggcgtgcctcaggatccacctgcagcagcctggagatcaggtctttgacagtgctggaacggtcatcccactcgggggaactgaactggtactggccctccatgatcatgcgtaacatcaggatctgccgccggtgccagaagggtggcgagccagccaggagtgtgaacaagatcaccccacaggcccagaggtcgacctccttgccatagcctgggtgggtttcatccatggagcatttaaggatctctggcgctagataccctggggtcccacacaactctcgaagcttctcgccaggttccaagtggcaggagaacccgaaatctgaaagtcggatctgcatattgtcatctaggagaatattctcgggcttcagatctcgatgcacaatgttgttggcatggagaaagctcactgcttccagcagagaccgcatgatggacctggtttccttttcagagagggccaccttctctgtgagatagtcaaacagctctcccttccgcatcaggtcaaacaccaggaacatgaagctagaagactcgtaggaatcgatgagggtgatgatgtgggggtggccggcgacctggcgaaggatgtgtgtctctcgccgtgtggcttcccgcacctcctccagctgctcaggactcagccgctcagctgtcacttccataatcttcaccgcaaactcgtggccagtagctcgatgaacacaacggcggaccacagagctcactcctctgccgatgacgtccttagggtcgtacttctggtaaaactctttggcggcggcccagtcgggcagctcatcctccggccccacgtccagcgtcatcctgaaggaggcgggggcctgagggggcaggcagaggagccagggtcgacgcgagctgcgctgtcgccgggtttgcctgcagtc

SEQ ID NO: 16546 - RNA, 1417 nt, Homo sapiens
  source 1..1417: mol_type = other RNA
gtgggctgggctgggctgggccatgtggcggcatgcaggagggacgtccacttgcaagcgtgaaggggctcagtctgtggggtgagcagcagctccatggtgggacacaggtgccctgccagccagcccttgtccctgaggagacctatggtgtctcaactctgctcaccttagaggccatctctgcctggctgcatcttcctccctggtggcagagagatctgaagggctcatctctgatgggggccagggacagcagcacggcccgcatggggagggggaacatagctgactcggcagcatgaccacaggtccatcattgggaatggtgagctcatgagtgctggccggtgggctggcgtccagacatccgggtgagggatggcatactgtccctggattgtgtaggcagcagacggaggtccggacacagcggcacagacgcccggtcgtcgggccatgcatccttcctcagtgcagagctccctcctctcgcacgtccctgctacaagcacatcctccagcatgaccacacagatctgcttgacgcactggatgatggcatctggggtccccgagatggtcaccgctcgctccgtggagttgggcagcatgtccccagccacctgcacctgggcacctgtggactccctgatctccttgatcttggagcctcctttgccgatcagggacccacactggctggcaggcaccaccagcctcagcgtcactgggggcttgctggtggcagggctgttgctcatggagttgatgatatcctcctcaaacttgtatgcgatcatggcaaaggccttgaagatggcgtctgtggggcctgtgatggtcacaatcctctctgggcagtttccctctgagatgttgatccttgcaccactctcctcacgcatcttcttcacagtttctcctttcttcccgatgatgcttccaacttcctttccatgcatcagcaggcggatggtgagggtcacattcaggccaccttctgagaccttggactccatccttctgccaaattgtggctgagggtggtggcttaaggtgctgagggtgctgtgaggaaggacagatggggcccagaaggcgtcaccttggaacaaagcagctctgtgaggctgggaacgatcaggtttgatgtgggtatcggacagatggccactctccccgtttagacaagatgagatgctcccactgagtccctcccatgacctgtaggaattgtgggagctacaattcaagatgagatttgggtggggacacagccagaccatatcagcatccatcaggaagacctcactgaagggggacctgggaacttcccccataagcaggctataaggtttagagcagatccatagacagcaaaggttcagacgtattgaactcagagcatcataac

SEQ ID NO: 16547 - RNA, 1384 nt, Homo sapiens
  source 1..1384: mol_type = other RNA
gtgggctgggctgggctgggccatgtggcggcatgcaggagggacgtccacttgcaagcgtgaaggggctcagtctgtggggtgagcagcagctccatggtgggacacaggtgccctgccagccagcccttgtccctgaggagacctatggtgtctcaactctgctcaccttagaggccatctctgcctggctgcatcttcctccctggtggcagagagatctgaagggctcatctctgatgggggccagggacagcagcacggcccgcatggggagggggaacatagctgactcggcagcatgaccacaggtccatcattgggaatggtgagctcatgagtgctggccggtgggctggcgtccagacatccgggtgagggatggcatactgtccctggattgtgtaggcctgaccacctgcaaaaatgacaggggtggaggcgggctttgggcggtagggaatggtggcacctttcggtggggactccagcatgaccacacagatctgcttgacgcactggatgatggcatctggggtccccgagatggtcaccgctcgctccgtggagttgggcagcatgtccccagccacctgcacctgggcacctgtggactccctgatctccttgatcttggagcctcctttgccgatcagggacccacactggctggcaggcaccaccagcctcagcgtcactgggggcttgctggtggcagggctgttgctcatggagttgatgatatcctcctcaaacttgtatgcgatcatggcaaaggccttgaagatggcgtctgtggggcctgtgatggtcacaatcctctctgggcagtttccctctgagatgttgatccttgcaccactctcctcacgcatcttcttcacagtttctcctttcttcccgatgatgcttccaacttcctttccatgcatcagcaggcggatggtgagggtcacattcaggccaccttctgagaccttggactccatccttctgccaaattgtggctgagggtggtggcttaaggtgctgagggtgctgtgaggaaggacagatggggcccagaaggcgtcaccttggaacaaagcagctctgtgaggctgggaacgatcaggtttgatgtgggtatcggacagatggccactctccccgtttagacaagatgagatgctcccactgagtccctcccatgacctgtaggaattgtgggagctacaattcaagatgagatttgggtggggacacagccagaccatatcagcatccatcaggaagacctcactgaagggggacctgggaacttcccccataagcaggctataaggtttagagcagatccatagacagcaaaggttcagacgtattgaactcagagcatcataac

SEQ ID NO: 16548 - RNA, 1453 nt, Homo sapiens
  source 1..1453: mol_type = other RNA
gtgggctgggctgggctgggccatgtggcggcatgcaggagggacgtccacttgcaagcgtgaaggggctcagtctgtggggtgagcagcagctccatggtgggacacaggtgccctgccagccagcccttgtccctgaggagacctatggtgtctcaactctgctcaccttagaggccatctctgcctggctgcatcttcctccctggtggcagagagatctgaagggctcatctctgatgggggccagggacagcagcacggcccgcatggggagggggaacatagctgactcggcagcatgaccacaggtccatcattgggaatggtgagctcatgagtgctggccggtgggctggcgtccagacatccgggtgagggatggcatactgtccctggattgtgtaggcgggcagcggcgggtgctgcagtaaaaggctgaggttggcagtggaggccgcgagcggatcggctcttacctgaccacctgcaaaaatgacaggggtggaggcgggctttgggcggtagggaatggtggcacctttcggtggggactccagcatgaccacacagatctgcttgacgcactggatgatggcatctggggtccccgagatggtcaccgctcgctccgtggagttgggcagcatgtccccagccacctgcacctgggcacctgtggactccctgatctccttgatcttggagcctcctttgccgatcagggacccacactggctggcaggcaccaccagcctcagcgtcactgggggcttgctggtggcagggctgttgctcatggagttgatgatatcctcctcaaacttgtatgcgatcatggcaaaggccttgaagatggcgtctgtggggcctgtgatggtcacaatcctctctgggcagtttccctctgagatgttgatccttgcaccactctcctcacgcatcttcttcacagtttctcctttcttcccgatgatgcttccaacttcctttccatgcatcagcaggcggatggtgagggtcacattcaggccaccttctgagaccttggactccatccttctgccaaattgtggctgagggtggtggcttaaggtgctgagggtgctgtgaggaaggacagatggggcccagaaggcgtcaccttggaacaaagcagctctgtgaggctgggaacgatcaggtttgatgtgggtatcggacagatggccactctccccgtttagacaagatgagatgctcccactgagtccctcccatgacctgtaggaattgtgggagctacaattcaagatgagatttgggtggggacacagccagaccatatcagcatccatcaggaagacctcactgaagggggacctgggaacttcccccataagcaggctataaggtttagagcagatccatagacagcaaaggttcagacgtattgaactcagagcatcataac

SEQ ID NO: 16549 - RNA, 1592 nt, Homo sapiens
  source 1..1592: mol_type = other RNA
gtgggctgggctgggctgggccatgtggcggcatgcaggagggacgtccacttgcaagcgtgaaggggctcagtctgtggggtgagcagcagctccatggtgggacacaggtgccctgccagccagcccttgtccctgaggagacctatggtgtctcaactctgctcaccttagaggccatctctgcctggctgcatcttcctccctggtggcagagagatctgaagggctcatctctgatgggggccagggacagcagcacggcccgcatggggagggggaacatagctgactcggcagcatgaccacaggtccatcattgggaatggtgagctcatgagtgctggccggtgggctggcgtccagacctgatgactggcccatcagattttgagcttcttcggaggagtgtaaaggcagcttttctccggggaaagcggggttggtctgtccgaggggaggaaagggggtttgctgcatggccaactggtggagcttggtcaactgatccgggtgagggatggcatactgtccctggattgtgtaggcgggcagcggcgggtgctgcagtaaaaggctgaggttggcagtggaggccgcgagcggatcggctcttacctgaccacctgcaaaaatgacaggggtggaggcgggctttgggcggtagggaatggtggcacctttcggtggggactccagcatgaccacacagatctgcttgacgcactggatgatggcatctggggtccccgagatggtcaccgctcgctccgtggagttgggcagcatgtccccagccacctgcacctgggcacctgtggactccctgatctccttgatcttggagcctcctttgccgatcagggacccacactggctggcaggcaccaccagcctcagcgtcactgggggcttgctggtggcagggctgttgctcatggagttgatgatatcctcctcaaacttgtatgcgatcatggcaaaggccttgaagatggcgtctgtggggcctgtgatggtcacaatcctctctgggcagtttccctctgagatgttgatccttgcaccactctcctcacgcatcttcttcacagtttctcctttcttcccgatgatgcttccaacttcctttccatgcatcagcaggcggatggtgagggtcacattcaggccaccttctgagaccttggactccatccttctgccaaattgtggctgagggtggtggcttaaggtgctgagggtgctgtgaggaaggacagatggggcccagaaggcgtcaccttggaacaaagcagctctgtgaggctgggaacgatcaggtttgatgtgggtatcggacagatggccactctccccgtttagacaagatgagatgctcccactgagtccctcccatgacctgtaggaattgtgggagctacaattcaagatgagatttgggtggggacacagccagaccatatcagcatccatcaggaagacctcactgaagggggacctgggaacttcccccataagcaggctataaggtttagagcagatccatagacagcaaaggttcagacgtattgaactcagagcatcataac

SEQ ID NO: 16550 - RNA, 1993 nt, Homo sapiens
  source 1..1993: mol_type = other RNA
gtgggctgggctgggctgggcccggtcctagccagcagagggcaggcgccctaggtcctggggaggctgcacatctcgcagtggcctgtgcctggctggttcatgaacgtgcagtgctgacaggcccacatggctgcagtggccgtgtgtgtggagcccccgacggcgccgtactcatggagacctgggagctgcccgccaactgtgcataaagatggcaacgccaggtgtggtggtacacatctgtaatcccagctactcgggaggtgcacagctgctcgatggtggcccactgctcagacctcttccatgtctgggcgagctcctcatttctggtccgcacggcctccagcagcaagctgatgctgtcctgcagaggcataacttcattggtgaccaggaacagcaagaggtggaaatctgagatggtatccaagaacacagatgaggtattctgagacaaataggtggccaagctatggaagtcctgtgtctcacccaatacatcccggttttcaataggaaatggattttgcgaaatagaaaaagtgtaaactggatccttggggaaagttgttgtgatgtctatgatgagatactccacaggcaggggccgggccagctgggtgatctcgttgccaaacttgtctacgtcctgtagccactgcagtaacaaacttggatccaaaatgtccgtctggagagagccggcacatgttgggatgcttgttctggaagtctcctgcagtgatgcactcttctgaacttaggaaataggtgtccttatttcgactgtagcggacggtaccctttcgggtatcttctgagacgaggtctgtaaatatccagccaaccttccgcaggccaagtttggcagcaatttcatcgaccacttcagcttttggatcctcaagaagctccaagctgttctgtgtaccaatctgaggtggctcataaatcgcagccacttcagccctgatgccaaggggaatgtctttgtgctccgtgtaccgtccgtataagtacccaaaatgctggttccctgtctttctccagaagtcaagaaagcggtcagcgacggtgtgattctcaaacatgatattgtccacatgcctgtacttctgtctgttcagcgtgatggcgctcggctggcacttagtacagatgccattcggccacgggaggtgcccctcgcaccctgacttaatcttgcagctgatgttctccagggcaacaaacttccccttgtcagcccctccagtcagcttccggatgtaggcgtggaaggacatgtgcttcacgggaggctcgagatggtttagatagtcctcatcgaatggctctagagggacgcagtgcacgcatttccccaaagggccgtggcggcatagctgtgggtctcggcttctgtaaatcttcccgtcctgtttgctgaggtactgatcaatctcatcctccaccacgttgggagcgccaaagactttgaagcccggtggaactgacgtctccatttcagatgagggcccagcaaggctcgagggaaacaggaacaacaaatcgccatgcttgatttttagcaagttgagggatttgttggaggaggctgttatctctccggtcttgtttctattgatgtaaaccgagaagccattattttggaagccaaactcctttgcaacctttttcaaaaatgttgctgctgtttctctctttgttgctgtgatccgcttcactccatccggggactggacacgaattatgatgctctcggccatggcggctgctcctgcctccgggctcgagccccgggccgccgccgcctgccgccccaagggcctcgcagacccggccgcggcctcagccccggccccggcctccctacgccgccgccaccgccgctccagcttcgcccgcccggctccgccagccgccgacgtcccggtgcctcgctcaatacgctcccctcgggcgcgaggccgggaaaccaggttcc

SEQ ID NO: 16551 - RNA, 2169 nt, Homo sapiens
  source 1..2169: mol_type = other RNA
gtgggctgggctgggctgggcccggtcctagccagcagagggcaggcgccctaggtcctggggaggctgcacatctcgcagtggcctgtgcctggctggttcatgaacgtgcagtgctgacaggcccacatggctgcagtggccgtgtgtgtggagcccccgacggcgccgtactcatggagacctgggagctgcccgccaactgtgcataaagatggcaacgccaggtgtggtggtacacatctgtaatcccagctactcgggaggtgcacagctgctcgatggtggcccactgctcagacctcttccatgtctgggcgagctcctcatttctggtccgcacggcctccagcagcaagctgatgctgtcctgcagaggcataacttcattggtgaccaggaacagcaagaggtggaaatctgagatggtatccaagaacacagatgaggtattctgagacaaataggtggccaagctatggaagtcctgtgtctcacccaatacatcccggttttcaataggaaatggattttgcgaaatagaaaaagtgtaaactggatccttggggaaagttgttgtgatgtctatgatgagatactccacaggcaggggccgggccagctgggtgatctcgttgccaaacttgtctacgtccttataaaacacatcaggcacgtactgctcactgctagactccttggcgtagccaagctccggggcgtccttgcatggcagcaaacactcatcacggaccagtgccatacactgattggacacctggtacccttcaaagtggacttggttgtcaggaccacctgcaagagagagacctgtagccactgcagtaacaaacttggatccaaaatgtccgtctggagagagccggcacatgttgggatgcttgttctggaagtctcctgcagtgatgcactcttctgaacttaggaaataggtgtccttatttcgactgtagcggacggtaccctttcgggtatcttctgagacgaggtctgtaaatatccagccaaccttccgcaggccaagtttggcagcaatttcatcgaccacttcagcttttggatcctcaagaagctccaagctgttctgtgtaccaatctgaggtggctcataaatcgcagccacttcagccctgatgccaaggggaatgtctttgtgctccgtgtaccgtccgtataagtacccaaaatgctggttccctgtctttctccagaagtcaagaaagcggtcagcgacggtgtgattctcaaacatgatattgtccacatgcctgtacttctgtctgttcagcgtgatggcgctcggctggcacttagtacagatgccattcggccacgggaggtgcccctcgcaccctgacttaatcttgcagctgatgttctccagggcaacaaacttccccttgtcagcccctccagtcagcttccggatgtaggcgtggaaggacatgtgcttcacgggaggctcgagatggtttagatagtcctcatcgaatggctctagagggacgcagtgcacgcatttccccaaagggccgtggcggcatagctgtgggtctcggcttctgtaaatcttcccgtcctgtttgctgaggtactgatcaatctcatcctccaccacgttgggagcgccaaagactttgaagcccggtggaactgacgtctccatttcagatgagggcccagcaaggctcgagggaaacaggaacaacaaatcgccatgcttgatttttagcaagttgagggatttgttggaggaggctgttatctctccggtcttgtttctattgatgtaaaccgagaagccattattttggaagccaaactcctttgcaacctttttcaaaaatgttgctgctgtttctctctttgttgctgtgatccgcttcactccatccggggactggacacgaattatgatgctctcggccatggcggctgctcctgcctccgggctcgagccccgggccgccgccgcctgccgccccaagggcctcgcagacccggccgcggcctcagccccggccccggcctccctacgccgccgccaccgccgctccagcttcgcccgcccggctccgccagccgccgacgtcccggtgcctcgctcaatacgctcccctcgggcgcgaggccgggaaaccaggttcc

SEQ ID NO: 16552 - RNA, 5528 nt, Homo sapiens
  source 1..5528: mol_type = other RNA
gtgggctgggctgggctgggcccggtcctagccagcagagggcaggcgccctaggtcctggggaggctgcacatctcgcagtggcctgtgcctggctggttcatgaacgtgcagtgctgacaggcccacatggctgcagtggccgtgtgtgtggagcccccgacggcgccgtactcatggagacctgggagctgcccgccaactgtgcctgggggtggtggtgcgcacctgtaatcccagctactaggaaggctgaggaaggagaatggcgtgaacctgggaggcggaggttgcagtgaaccgaggttgcagtaagccgagatctcaaaacaaacaaacaaacaaacaacaacaacaaaaaacctacctaggaatgaatctgccggcccacagggtaatgaattgtgtgctgaactttctaagaccctgagacacagttctcgcgagggtggcacggttttgcctcccactcgcaaggtacgagagtcccagctgcttcacatcttcactcacacttgacattgtcgcgtttttttcatttcagccacactgatgaatgtgtaacggcttctcatgttttaatttgcatttccctgatgactaatgatagtgactgttcctgcatctccttttttttgttgttgccgaggctggagtgcaatggcgcaatctcggctcgctgcaacctctgcctcctgggttcaagcgattctcctacctcagcctcccaagtagctaggattacaggcacgtgccaccacacctggctaattttttttatttttagtagagatgggttttcaccatgttggcctggctgtctcgaactcctgacctcaaatgatccaccgcctcggcctcccaaagtgctgggattacaggcgtgagctaccatgcccgacctgcatttccttttgtgaaacgtttcaccctccgcccagcttcttcttctgctttctgtttgattaacaacaggcagagttatttttaagtttcagatagaagtcatgttgtgtgtatgtactgctaatactgcgtcccccattggtgccttttcatgtttctaacagtgccctgtgatgagcacaagtgttttgtttagataaatttatttatcaatttacctatttttatgccagtgtttttctgtgttctaccccaaggtcctgcatcctgcctaaaagaatctttgcgtaccccaaggccctgaagagattcaacttaataactgttttacagtttttatttttttaagacagggtattgctctgtcattcaggctggagtggtataatcatggctcactgtgacctcgacctcctgactcatgggatcctcccatttcagcctccccagaagctgggattataggcgtggaccactcaccatgcccagctaattcttttttttttaatattgtttttttgtacagacggggcttcactatgctgtgtgggctggtctcacacttctgggctacagtgtcctccagctttggcctcctagagtgttaggattatagctatgagacatcatgcccagcctgcttcatagttttaccttttaccattaggcctatgacccatcctgagctgatctttgtgtcttgtgtatacacgtctgtaatcccagcactttgggagaccgaggcaggtggatcacctgaggtcaggagttccagaccagcctgaccaacatggtgaaaccccatctctactaaaaatataaaaattagccaggcgtgggtgcacgcctgtagtcccagctactcgggaggctgaggcaggagtatcacttgaacccaggacgtggaggttgcagtaagtggagatcatgagattgcactgcagcctgggtgacagggtgagattccgtctcaaaacaaaacaaaacaacccatgagggccgggcgcggtggctcacacctataatcccagcactttgggaagccgaggtgggtggatcacttgaggtcaggagtttgagaccagcctggccaacatggagaaaccctgtctctactaaaactaaaaaaattagctgggtgtggtggcagccacctgtaattccagctacttaggaggcagaggctggacaatggcttgaacccgggaggtggaggctgcagtgagctgagatcacactactgcactccagcctgggcaacagaacaagactttgtctcaaaacaaacaaacaaaaaacccatgaaaaaatgcccaacatcactaatcatcagagatgcaaattaaaaccacagtgagataccagtcagaacttacaccagtcagaactgcctattattaaagagttggctggacatggtggcttaccactgcaatctcagcactgaggcgggaggatcgcttgggcccaagagttcaagaccagcctgggcaacatagtgagacctcatctctacaacaaatttaaaaaatcagccagggatggtggcacatgcttgtagtcccagctgctcaggaggctgaggcgggaggattgtttgagcctggggaggtcaaggtgagactgacctcaaatgccactgcacttcagcctgggtgacagagtgagaacctgtctcaaaaaaaaaaggaggggggaaaaaaaaaaggtcaggtgcagtggctcacagctgtaatctcagcactttgggaaccaaggcaggaagatcacttgagcctaggagtttgagaccagcctgggcaacatggcaagaccacatcttttttttttttttgagacagagtcttgctctgtcgcccaggctggagtacagtggcacgatctcagctcactacaacctacgcttcctgggtcaagtgattctcctgcctcagcctcctgagtagctgggattacaggcgctcgccaccatgcccagctaatttttgtagttttaacagaaatggggtttcaccatgttggccaggatggtctcaatcccttgacgttgtgatccacctgcctcagcctcccaaagtgctgggattacaggtgtgagccagccaccgggcccggccaaccctatctcttaaagaaaaaaaaaaaacaccaaccaaaaacattagttgggtgtagtggctcatgtttatactcctaggtactccgaaagctgatgcaggaggatcgcttgagctcaggaattgaaggctgtagtgagctatgatcactccactgcactccagcctaggcaacagagtgaaaccctgtctctaaaagggaaacaaaaaagaaaaaaaaaaaaaagactggtgtcattgttagaactgcatcaaagggctgggtgcagtggctcccaggtataatctcaggactttgtgaggctgaggtgcaaggaatgcttgaggccaaagtttgagaccagtctgggcaacacagtgagacctcattgatacaaaaatattaaaaaattttgcagccataaaaaggaatgaaatcatgtcctttgcagcaacatggatgcagttgaaggccattattctaagcaaactaatgcaggaacagcaaaccaaatactacatgttttcatttataagtgggagctaaacatgggtactcacgtacataaagatggcaacgccaggtgtggtggtacacatctgtaatcccagctactcgggaggtgcacagctgctcgatggtggcccactgctcagacctcttccatgtctgggcgagctcctcatttctggtccgcacggcctccagcagcaagctgatgctgtcctgcagaggcataacttcattggtgaccaggaacagcaagaggtggaaatctgagatggtatccaagaacacagatgaggtattctgagacaaataggtggccaagctatggaagtcctgtgtctcacccaatacatcccggttttcaataggaaatggattttgcgaaatagaaaaagtgtaaactggatccttggggaaagttgttgtgatgtctatgatgagatactccacaggcaggggccgggccagctgggtgatctcgttgccaaacttgtctacgtccttataaaacacatcaggcacgtactgctcactgctagactccttggcgtagccaagctccggggcgtccttgcatggcagcaaacactcatcacggaccagtgccatacactgattggacacctggtacccttcaaagtggacttggttgtcaggaccacctgcaagagagagacctgtagccactgcagtaacaaacttggatccaaaatgtccgtctggagagagccggcacatgttgggatgcttgttctggaagtctcctgcagtgatgcactcttctgaacttaggaaataggtgtccttatttcgactgtagcggacggtaccctttcgggtatcttctgagacgaggtctgtaaatatccagccaaccttccgcaggccaagtttggcagcaatttcatcgaccacttcagcttttggatcctcaagaagctccaagctgttctgtgtaccaatctgaggtggctcataaatcgcagccacttcagccctgatgccaaggggaatgtctttgtgctccgtgtaccgtccgtataagtacccaaaatgctggttccctgtctttctccagaagtcaagaaagcggtcagcgacggtgtgattctcaaacatgatattgtccacatgcctgtacttctgtctgttcagcgtgatggcgctcggctggcacttagtacagatgccattcggccacgggaggtgcccctcgcaccctgacttaatcttgcagctgatgttctccagggcaacaaacttccccttgtcagcccctccagtcagcttccggatgtaggcgtggaaggacatgtgcttcacgggaggctcgagatggtttagatagtcctcatcgaatggctctagagggacgcagtgcacgcatttccccaaagggccgtggcggcatagctgtgggtctcggcttctgtaaatcttcccgtcctgtttgctgaggtactgatcaatctcatcctccaccacgttgggagcgccaaagactttgaagcccggtggaactgacgtctccatttcagatgagggcccagcaaggctcgagggaaacaggaacaacaaatcgccatgcttgatttttagcaagttgagggatttgttggaggaggctgttatctctccggtcttgtttctattgatgtaaaccgagaagccattattttggaagccaaactcctttgcaacctttttcaaaaatgttgctgctgtttctctctttgttgctgtgatccgcttcactccatccggggactggacacgaattatgatgctctcggccatggcggctgctcctgcctccgggctcgagccccgggccgccgccgcctgccgccccaagggcctcgcagacccggccgcggcctcagccccggccccggcctccctacgccgccgccaccgccgctccagcttcgcccgcccggctccgccagccgccgacgtcccggtgcctcgctcaatacgctcccctcgggcgcgaggccgggaaaccaggttcc

SEQ ID NO: 16553 - RNA, 672 nt, Homo sapiens
  source 1..672: mol_type = other RNA
gtgggctgggctgggctgggcccggtcctagccagcagagggcaggcgccctaggtcctggggaggctgcacatctcgcagtggcctgtgcctggctggttcatgaacgtgcagtgctgacaggcccacatggctgcagtggccgtgtgtgtggagcccccgacggcgccgtactcatggagacctgggagctgcccgccaactgtgctgcacagctgctcgatggtggcccactgctcagacctcttccatgtctgggcgagctcctcatttctggtccgcacggcctccagcagcaagctgatgctgtcctgcagaggcataacttcattggtgaccaggaacagcaagaggtggaaatctgagatggtatccaagaacacagatgaggtattctgagacaaataggtggccaagctatggaagtcctgtgtctcacccaatacatcccggttttcaataggaaatggattttgcgaaatagaaaaagtgtaaactggatccttggggaaagttgttgtgatgtctatgatgagatactccacaggcaggggccgggccagctgggtgatctcgttgccaaacttgtctacgtcctctttagagcagccatccttggagttgctcaacgccctcttctcttctccctctgaaccacagcttggctcatct

SEQ ID NO: 16554 - RNA, 1934 nt, Homo sapiens
  source 1..1934: mol_type = other RNA
gtgggctgggctgggctgggcccggtcctagccagcagagggcaggcgccctaggtcctggggaggctgcacatctcgcagtggcctgtgcctggctggttcatgaacgtgcagtgctgacaggcccacatggctgcagtggccgtgtgtgtggagcccccgacggcgccgtactcatggagacctgggagctgcccgccaactgtgctgcacagctgctcgatggtggcccactgctcagacctcttccatgtctgggcgagctcctcatttctggtccgcacggcctccagcagcaagctgatgctgtcctgcagaggcataacttcattggtgaccaggaacagcaagaggtggaaatctgagatggtatccaagaacacagatgaggtattctgagacaaataggtggccaagctatggaagtcctgtgtctcacccaatacatcccggttttcaataggaaatggattttgcgaaatagaaaaagtgtaaactggatccttggggaaagttgttgtgatgtctatgatgagatactccacaggcaggggccgggccagctgggtgatctcgttgccaaacttgtctacgtcctgtagccactgcagtaacaaacttggatccaaaatgtccgtctggagagagccggcacatgttgggatgcttgttctggaagtctcctgcagtgatgcactcttctgaacttaggaaataggtgtccttatttcgactgtagcggacggtaccctttcgggtatcttctgagacgaggtctgtaaatatccagccaaccttccgcaggccaagtttggcagcaatttcatcgaccacttcagcttttggatcctcaagaagctccaagctgttctgtgtaccaatctgaggtggctcataaatcgcagccacttcagccctgatgccaaggggaatgtctttgtgctccgtgtaccgtccgtataagtacccaaaatgctggttccctgtctttctccagaagtcaagaaagcggtcagcgacggtgtgattctcaaacatgatattgtccacatgcctgtacttctgtctgttcagcgtgatggcgctcggctggcacttagtacagatgccattcggccacgggaggtgcccctcgcaccctgacttaatcttgcagctgatgttctccagggcaacaaacttccccttgtcagcccctccagtcagcttccggatgtaggcgtggaaggacatgtgcttcacgggaggctcgagatggtttagatagtcctcatcgaatggctctagagggacgcagtgcacgcatttccccaaagggccgtggcggcatagctgtgggtctcggcttctgtaaatcttcccgtcctgtttgctgaggtactgatcaatctcatcctccaccacgttgggagcgccaaagactttgaagcccggtggaactgacgtctccatttcagatgagggcccagcaaggctcgagggaaacaggaacaacaaatcgccatgcttgatttttagcaagttgagggatttgttggaggaggctgttatctctccggtcttgtttctattgatgtaaaccgagaagccattattttggaagccaaactcctttgcaacctttttcaaaaatgttgctgctgtttctctctttgttgctgtgatccgcttcactccatccggggactggacacgaattatgatgctctcggccatggcggctgctcctgcctccgggctcgagccccgggccgccgccgcctgccgccccaagggcctcgcagacccggccgcggcctcagccccggccccggcctccctacgccgccgccaccgccgctccagcttcgcccgcccggctccgccagccgccgacgtcccggtgcctcgctcaatacgctcccctcgggcgcgaggccgggaaaccaggttcc

SEQ ID NO: 16555 - RNA, 2074 nt, Homo sapiens
  source 1..2074: mol_type = other RNA
gtgggctgggctgggctgggcccggtcctagccagcagagggcaggcgccctaggtcctggggaggctgcacatctcgcagtggcctgtgcctggctggttcatgaacgtgcagtgctgacaggcccacatggctgcagtggccgtgtgtgtggagcccccgacggcgccgtactcatggagacctgggagctgcccgccaactgtgctgcacagctgctcgatggtggcccactgctcagacctcttccatgtctgggcgagctcctcatttctggtccgcacggcctccagcagcaagctgatgctgtcctgcagaggcataacttcattggtgaccaggaacagcaagaggtggaaatctgagatggtatccaagaacacagatgaggtattctgagacaaataggtggccaagctatggaagtcctgtgtctcacccaatacatcccggttttcaataggaaatggattttgcgaaatagaaaaagtgtaaactggatccttggggaaagttgttgtgatgtctatgatgagatactccacaggcaggggccgggccagctgggtgatctcgttgccaaacttgtctacgtccttataaaacacatcaggcacgtactgctcactgctagactccttggcgtagccaagctccggggcgtccttgcatggcagcaaacactcatcacggaccagtgccatacactgattggacacctggtacccttcaaagtggacttggttgtcaggaccacctgcaagagagagacctgtagccactgcagtaacaaacttggatccaaaatgtccgtctggagagagccggcacatgttgggatgcttgttctggaagtctcctgcagtgatgcactcttctgaacttaggaaataggtgtccttatttcgactgtagcggacggtaccctttcgggtatcttctgagacgaggtctgtaaatatccagccaaccttccgcaggccaagtttggcagcaatttcatcgaccacttcagcttttggatcctcaagaagctccaagctgttctgtgtaccaatctgaggtggctcataaatcgcagccacttcagccctgatgccaaggggaatgtctttgtgctccgtgtaccgtccgtataagtacccaaaatgctggttccctgtctttctccagaagtcaagaaagcggtcagcgacggtgtgattctcaaacatgatattgtccacatgcctgtacttctgtctgttcagcgtgatggcgctcggctggcacttagtacagatgccattcggccacgggaggtgcccctcgcaccctgacttaatcttgcagctgatgttctccagggcaacaaacttccccttgtcagcccctccagtcagcttccggatgtaggcgtggaaggacatgtgcttcacgggaggctcgagatggtttagatagtcctcatcgaatggctctagagggacgcagtgcacgcatttccccaaagggccgtggcggcatagctgtgggtctcggcttctgtaaatcttcccgtcctgtttgctgaggtactgatcaatctcatcctccaccacgttgggagcgccaaagactttgaagcccggtggaactgacgtctccatttcagatgagggcccagcaaggctcgagggaaacaggaacaacaaatcgccatgcttgatttttagcaagttgagggatttgttggaggaggctgttatctctccggtcttgtttctattgatgtaaaccgagaagccattattttggaagccaaactcctttgcaacctttttcaaaaatgttgctgctgtttctctctttgttgctgtgatccgcttcactccatccggggactggacacgaattatgatgctctcggccatggcggctgctcctgcctccgggctcgagccccgggccgccgccgcctgccgccccaagggcctcgcagacccggccgcggcctcagccccggccccggcctccctacgccgccgccaccgccgctccagcttcgcccgcccggctccgccagccgccgacgtcccggtgcctcgctcaatac

SEQ ID NO: 16556 - RNA, 2059 nt, Homo sapiens
  source 1..2059: mol_type = other RNA
gtgggctgggctgggctgggcccggtcctagccagcagagggcaggcgccctaggtcctggggaggctgcacatctcgcagtggcctgtgcctggctggttcatgaacgtgcagtgctgacaggcccacatggctgcagtggccgtgtgtgtggagcccccgacggcgccgtactcatggagacctgggagctgcccgccaactgtgctgcacagctgctcgatggtggcccactgctcagacctcttccatgtctgggcgagctcctcatttctggtccgcacggcctccagcagcaagctgatgctgtcctgcagaggcataacttcattggtgaccaggaacagcaagaggtggaaatctgagatggtatccaagaacacagatgaggtattctgagacaaataggtggccaagctatggaagtcctgtgtctcacccaatacatcccggttttcaataggaaatggattttgcgaaatagaaaaagtgtaaactggatccttggggaaagttgttgtgatgtctatgatgagatactccacaggcaggggccgggccagctgggtgatctcgttgccaaacttgtctacgtccttataaaacacatcaggcacgtactgctcactgctagactccttggcgtagccaagctccggggcgtccttgcatggcagcaaacactcatcacggaccagtgccatacactgattggacacctggtacccttcaaagtggacttggttgtcaggaccacctgtagccactgcagtaacaaacttggatccaaaatgtccgtctggagagagccggcacatgttgggatgcttgttctggaagtctcctgcagtgatgcactcttctgaacttaggaaataggtgtccttatttcgactgtagcggacggtaccctttcgggtatcttctgagacgaggtctgtaaatatccagccaaccttccgcaggccaagtttggcagcaatttcatcgaccacttcagcttttggatcctcaagaagctccaagctgttctgtgtaccaatctgaggtggctcataaatcgcagccacttcagccctgatgccaaggggaatgtctttgtgctccgtgtaccgtccgtataagtacccaaaatgctggttccctgtctttctccagaagtcaagaaagcggtcagcgacggtgtgattctcaaacatgatattgtccacatgcctgtacttctgtctgttcagcgtgatggcgctcggctggcacttagtacagatgccattcggccacgggaggtgcccctcgcaccctgacttaatcttgcagctgatgttctccagggcaacaaacttccccttgtcagcccctccagtcagcttccggatgtaggcgtggaaggacatgtgcttcacgggaggctcgagatggtttagatagtcctcatcgaatggctctagagggacgcagtgcacgcatttccccaaagggccgtggcggcatagctgtgggtctcggcttctgtaaatcttcccgtcctgtttgctgaggtactgatcaatctcatcctccaccacgttgggagcgccaaagactttgaagcccggtggaactgacgtctccatttcagatgagggcccagcaaggctcgagggaaacaggaacaacaaatcgccatgcttgatttttagcaagttgagggatttgttggaggaggctgttatctctccggtcttgtttctattgatgtaaaccgagaagccattattttggaagccaaactcctttgcaacctttttcaaaaatgttgctgctgtttctctctttgttgctgtgatccgcttcactccatccggggactggacacgaattatgatgctctcggccatggcggctgctcctgcctccgggctcgagccccgggccgccgccgcctgccgccccaagggcctcgcagacccggccgcggcctcagccccggccccggcctccctacgccgccgccaccgccgctccagcttcgcccgcccggctccgccagccgccgacgtcccggtgcctcgctcaatac

SEQ ID NO: 16557 - RNA, 443 nt, Homo sapiens
  source 1..443: mol_type = other RNA
gtgggctgggctgggctgggcccggtcctagccagcagagggcaggcgccctaggtcctggggaggctgcacatctcgcagtggcctgtgcctggctggttcatgaacgtgcagtgctgacaggcccacatggctgcagtggccgtgtgtgtggagcccccgacggcgccgtactcatggagacctgggagctgcccgccaactgtgctgcacagctgctcgatggtggcccactgctcagacctcttccatgtctgggcgagctcctcatttctggtccgcacggcctccagcagcaagctgatgctgtcctttcaccacctgtccagacagatgggcagcagctgaacctcggagcaggaggtgcagttccctgggctgactagggaaggcacaggcagggaagaggcacagggtgcctgatgtcaaatacccgagtgagt

SEQ ID NO: 16558 - RNA, 2639 nt, Homo sapiens
  source 1..2639: mol_type = other RNA
gtgggctgggctgggctgggccctctatctcacagggcctgagtcaagccagcccgccctgcaaggcaggggctgacctgcaagcggagatctcacttcctcttaccccaaattcatacctccattttccccgcccccatctctccccagggtcctcaagtgggaaagggagaggtagcatccctcggatccaggcccactccactccgtctccggcaccagtgggcaggctgagtctgggcctcaaggggccctgggcttagggtatctatggcagtaggaaaatgacatggacaggctcttcaggggtaggctaaagtcctctggccagcagtacccagagaaaatgggcagcagcaggtaaaccagccaggaggtggagtcctctgaacccacagcagaccccaccctcctgcccagcccctgcccacattgggggtcaggaccactgagactctggtcaggacagtgggtgctctcagcagtgtggcaagctcagagcagagctcccaaggaccataccacactggttcaaaacccataggtgacaccatcccagcagaagcttccatgggtgctggatcccagggctgcatcctgagcacaggtgggcagactggaacataacactaggacccaagggatccagaacattttaggcccatctcctgggctgctccagcctgttgccatgacttgggcagtgagtgggcctcctgccaggtggcagggcacagcttagaccaaacccttggcctcccccctctgcagctacctctgaccaagaaggaactagcaagcctatgctggcaagaccataggtggggtgctgggaatcctcggggccggctggcacccactcctggtgctcaagggagagacccacttgttcagatgcataggcctcaggcggttcaaggcagtcttagagccacagagtcaaataaaaatcaattttgagagaccacagcacctgctgctttgatcgtgatgttcaaggcaagttgcaagtcaaggcaagtgtcccagaggccctgggcagctgagtgcacctgtgtttgatcttcccctgatgatggacactcccagctgaccatccaaacaccaggaaaacatccccctttcctgggctcagttcctagtctacttgctggtacgaacccaacccacacactccccgcccacaatgcagctccttccaaatcctcccacaagccacctttgtgggacttggaagctgcttaggatgggccctgccctctgcgggaagccaatcctagcagaaaggtaagctaaacaacagtctcagaatctgagacccagtgactgttccccccgccccaggccttgggcctgaagtgggggcctgcctgtggcctctgtggtgggctcactcccacccccaacagtggccccaggagaggctttcccaagagtcttcaaactccacccaccccagccctagcatcagggactccccaccccccactggagtgttaatatcattaatgtacaaataagatccaaagatataccaaagatcgagaaacagctggctccgacctccctcccacagagccttcccagggttagctgaaaaagagccctttggcatctacagaagccagtcggagtttatggtttcatttgcccaaaaatacacctttggggacctcaaattctttccaagaatcactaccacacatatgaatttgaacattcgccacccttccaccatccatttctcgcaggaacttcaaaataaaaatggccagtctgcccccactctggctcctcgtctatggctgtctcttcttttccaggggctgcagttctgatgtgaatgatggtgccattccagcattgggcctctggcaggctgcatcacatgatggcacagcatgagttttgtttccgggcagttttatagaaggctttagactgtgttcccagcacctcggatttggacaccaagtcatctagcttctcacctcgctctaacagagactccatggtgttgtgcagaatgattttggtctcatctagttcggcctgcactttagtcatgggatcagcttctcgtgggttctggtatctactgaggtgaccatccagggctgggtaatggattgtagcaggggatcctactggccagtctatcctgtcgacttgcttggagaattcatctagtaccttctccagcaaggtaaaggccacccgggatgggtattcattgtcagcaatgaccacacctgcaagactatcattccggacgtagacgtggcacagatagtcttgttctttgacagaagctctagtgcctttcgatgagcgctccacaatcagttgactcgtgaaggtcatgaattcctgaacgctggatctctggaaaaagctgaaggaagacacatcgtatgcggctttgagcagcaccaccttggcctcgcctttgtagaggacgctgaggctgtacagcttcatggctccgcgccctcaggccgcccgcctgcccagctgcgggacccgttctcagggagcagcgcggccgccgcccctcgggaccgccgccgcctaccggcctctcagcagccggctgctgacggggccaccgccggcttcctcctcctggctcgcaatcc

SEQ ID NO: 16559 - RNA, 2537 nt, Homo sapiens
  source 1..2537: mol_type = other RNA
gtgggctgggctgggctgggccctctatctcacagggcctgagtcaagccagcccgccctgcaaggcaggggctgacctgcaagcggagatctcacttcctcttaccccaaattcatacctccattttccccgcccccatctctccccagggtcctcaagtgggaaagggagaggtagcatccctcggatccaggcccactccactccgtctccggcaccagtgggcaggctgagtctgggcctcaaggggccctgggcttagggtatctatggcagtaggaaaatgacatggacaggctcttcaggggtaggctaaagtcctctggccagcagtacccagagaaaatgggcagcagcaggtaaaccagccaggaggtggagtcctctgaacccacagcagaccccaccctcctgcccagcccctgcccacattgggggtcaggaccactgagactctggtcaggacagtgggtgctctcagcagtgtggcaagctcagagcagagctcccaaggaccataccacactggttcaaaacccataggtgacaccatcccagcagaagcttccatgggtgctggatcccagggctgcatcctgagcacaggtgggcagactggaacataacactaggacccaagggatccagaacattttaggcccatctcctgggctgctccagcctgttgccatgacttgggcagtgagtgggcctcctgccaggtggcagggcacagcttagaccaaacccttggcctcccccctctgcagctacctctgaccaagaaggaactagcaagcctatgctggcaagaccataggtggggtgctgggaatcctcggggccggctggcacccactcctggtgctcaagggagagacccacttgttcagatgcataggcctcaggcggttcaaggcagtcttagagccacagagtcaaataaaaatcaattttgagagaccacagcacctgctgctttgatcgtgatgttcaaggcaagttgcaagtcaaggcaagtgtcccagaggccctgggcagctgagtgcacctgtgtttgatcttcccctgatgatggacactcccagctgaccatccaaacaccaggaaaacatccccctttcctgggctcagttcctagtctacttgctggtacgaacccaacccacacactccccgcccacaatgcagctccttccaaatcctcccacaagccacctttgtgggacttggaagctgcttaggatgggccctgccctctgcgggaagccaatcctagcagaaaggtaagctaaacaacagtctcagaatctgagacccagtgactgttccccccgccccaggccttgggcctgaagtgggggcctgcctgtggcctctgtggtgggctcactcccacccccaacagtggccccaggagaggctttcccaagagtcttcaaactccacccaccccagccctagcatcagggactccccaccccccactggagtgttaatatcattaatgtacaaataagatccaaagatataccaaagatcgagaaacagctggctccgacctccctcccacagagccttcccagggttagctgaaaaagagccctttggcatctacagaagccagtcggagtttatggtttcatttgcccaaaaatacacctttggggacctcaaattctttccaagaatcactaccacacatatgaatttgaacattcgccacccttccaccatccatttctcgcaggaacttcaaaataaaaatggccagtctgcccccactctggctcctcgtctatggctgtctcttcttttccaggggctgcagttctgatgtgaatgatggtgccattccagcattgggcctctggcaggctgcatcacatgatggcacagcatgagttttgtttccgggccagaatgattttggtctcatctagttcggcctgcactttagtcatgggatcagcttctcgtgggttctggtatctactgaggtgaccatccagggctgggtaatggattgtagcaggggatcctactggccagtctatcctgtcgacttgcttggagaattcatctagtaccttctccagcaaggtaaaggccacccgggatgggtattcattgtcagcaatgaccacacctgcaagactatcattccggacgtagacgtggcacagatagtcttgttctttgacagaagctctagtgcctttcgatgagcgctccacaatcagttgactcgtgaaggtcatgaattcctgaacgctggatctctggaaaaagctgaaggaagacacatcgtatgcggctttgagcagcaccaccttggcctcgcctttgtagaggacgctgaggctgtacagcttcatggctccgcgccctcaggccgcccgcctgcccagctgcgggacccgttctcagggagcagcgcggccgccgcccctcgggaccgccgccgcctaccggcctctcagcagccggctgctgacggggccaccgccggcttcctcctcctggctcgcaatcc

SEQ ID NO: 16560 - RNA, 2690 nt, Homo sapiens
  source 1..2690: mol_type = other RNA
gtgggctgggctgggctgggccctctatctcacagggcctgagtcaagccagcccgccctgcaaggcaggggctgacctgcaagcggagatctcacttcctcttaccccaaattcatacctccattttccccgcccccatctctccccagggtcctcaagtgggaaagggagaggtagcatccctcggatccaggcccactccactccgtctccggcaccagtgggcaggctgagtctgggcctcaaggggccctgggcttagggtatctatggcagtaggaaaatgacatggacaggctcttcaggggtaggctaaagtcctctggccagcagtacccagagaaaatgggcagcagcaggtaaaccagccaggaggtggagtcctctgaacccacagcagaccccaccctcctgcccagcccctgcccacattgggggtcaggaccactgagactctggtcaggacagtgggtgctctcagcagtgtggcaagctcagagcagagctcccaaggaccataccacactggttcaaaacccataggtgacaccatcccagcagaagcttccatgggtgctggatcccagggctgcatcctgagcacaggtgggcagactggaacataacactaggacccaagggatccagaacattttaggcccatctcctgggctgctccagcctgttgccatgacttgggcagtgagtgggcctcctgccaggtggcagggcacagcttagaccaaacccttggcctcccccctctgcagctacctctgaccaagaaggaactagcaagcctatgctggcaagaccataggtggggtgctgggaatcctcggggccggctggcacccactcctggtgctcaagggagagacccacttgttcagatgcataggcctcaggcggttcaaggcagtcttagagccacagagtcaaataaaaatcaattttgagagaccacagcacctgctgctttgatcgtgatgttcaaggcaagttgcaagtcaaggcaagtgtcccagaggccctgggcagctgagtgcacctgtgtttgatcttcccctgatgatggacactcccagctgaccatccaaacaccaggaaaacatccccctttcctgggctcagttcctagtctacttgctggtacgaacccaacccacacactccccgcccacaatgcagctccttccaaatcctcccacaagccacctttgtgggacttggaagctgcttaggatgggccctgccctctgcgggaagccaatcctagcagaaaggtaagctaaacaacagtctcagaatctgagacccagtgactgttccccccgccccaggccttgggcctgaagtgggggcctgcctgtggcctctgtggtgggctcactcccacccccaacagtggccccaggagaggctttcccaagagtcttcaaactccacccaccccagccctagcatcagggactccccaccccccactggagtgttaatatcattaatgtacaaataagatccaaagatataccaaagatcgagaaacagctggctccgacctccctcccacagagccttcccagggttagctgaaaaagagccctttggcatctacagaagccagtcggagtttatggtttcatttgcccaaaaatacacctttggggacctcaaattctttccaagaatcactaccacacatatgaatttgaacattcgccacccttccaccatccatttctcgcaggaacttcaaaataaaaatggccagtctgcccccactctggctcctcgtctatggctgtctcttcttttccaggggctgcagttctgatgtgaatgatggtgccattccagcattgggcctctggcaggctgcatcacatgatggcacagcatgagttttgtttccgggcctgagagaaagcggcagtcagcagcacccatccttgtcaattaaatattttagttttatagaaggctttagactgtgttcccagcacctcggatttggacaccaagtcatctagcttctcacctcgctctaacagagactccatggtgttgtgcagaatgattttggtctcatctagttcggcctgcactttagtcatgggatcagcttctcgtgggttctggtatctactgaggtgaccatccagggctgggtaatggattgtagcaggggatcctactggccagtctatcctgtcgacttgcttggagaattcatctagtaccttctccagcaaggtaaaggccacccgggatgggtattcattgtcagcaatgaccacacctgcaagactatcattccggacgtagacgtggcacagatagtcttgttctttgacagaagctctagtgcctttcgatgagcgctccacaatcagttgactcgtgaaggtcatgaattcctgaacgctggatctctggaaaaagctgaaggaagacacatcgtatgcggctttgagcagcaccaccttggcctcgcctttgtagaggacgctgaggctgtacagcttcatggctccgcgccctcaggccgcccgcctgcccagctgcgggacccgttctcagggagcagcgcggccgccgcccctcgggaccgccgccgcctaccggcctctcagcagccggctgctgacggggccaccgccggcttcctcctcctggctcgcaatcc

SEQ ID NO: 16561 - RNA, 473 nt, Homo sapiens
  source 1..473: mol_type = other RNA
gtgggctgggctgggctgggccgggccaggcgcgatggcagggttctctccttggcggcggcggcagcggcggaggcggcggcggcggcgggcgaggcagcccttcgcgggcagcaccagaactggtcggtgatttaggtagtttcctgttgttgggatccacctttctctcgacagcacgacactgccttcattacttcagttgaaatcgtctccaggtacctctgcgcgcgggggtcgggccgggcggggcatcacggccctggtcgtgccaggcctgcggtggcaacctcggctttccctgctcaggagcctcgtgtctttctccgcagcgctttgccagccggccggctttccccttccaccacacacctccacccttctctctgtaagctcggccgctgctaggagtcgcctctcttttcttccttcttttccctgtcttcccttcctcttttatctcttctttcttt

SEQ ID NO: 16562 - RNA, 62 nt, Homo sapiens
  source 1..62: mol_type = other RNA
gtgggctgggctgggctgggccgggccgaccggccgccgcctccccgcctcaccgggccgct

SEQ ID NO: 16563 - RNA, 79 nt, Homo sapiens
  source 1..79: mol_type = other RNA
gtgggctgggctgggctgggccgggccgggagcgagtgcgcgccgacagctgatcgggcagccgcctggctcgcctttc

SEQ ID NO: 16564 - RNA, 2154 nt, Homo sapiens
  source 1..2154: mol_type = other RNA
gtgggctgggctgggctgggcctaaaggtttccccgcgctcacgttcacgttcacgttcatgttcacgctcattatctttgtcatccccaaagtggattttctggtgctcaatcagggcagaactatgaaggaaggtttccttacacaccctgcactcgtagaatttgtctttgccatatattttctgaagctcactaaaggtggggctaggcatgaaggcttcctcacattcctgattcttacattccacaagataacctctagcatgaatcttccgatgttcagccaaggcggcactcttattgaaggtctctccacagtccttacattcaaaacgtttccctccaacctgacttttctgaacttcactgacagccacactgtggataaaggactcaccatactcatagaggttctctctagtatgcatgatctggtgctcaacaaattctgagatgacactgaacgacctcccacactcatcacatacatatggcattgccccaaaatcaattggctgtgactcggtaaaggagggggagctgaggctgctcaggctgctcacgctcatggcttttctcatctcactaccacattcaaagggcttcttcctgggacagcctttttgatcgtgaatcgagcccttcccatctgtgtcaaaatgatagcgcctctttctttcaagaactctctttctggaaacaagggttgaattaaacctaaagcctcccctaaatgcattcccttcataaacccgctgctggatcactgactccctcttgttcaatgaaatgtccttccagttatcatctgacattctggggaatctctgtgaccggtcgcttgactcccttgctcttcccgatttggaactgcgtgacacatccttgatgaatttttccattatcactccgtgggaagattcatcttcacaaatcccccgccggtgggttgattttttggcttcaggcatagtttttagaccgagggagagcagcttcctgtagttttccatgttgtcctggattgtgttgtgaggtttcctgtcctcagcgaggtccaccacattttggtatgattcagcatcctgagatcgggactcataagccctggagtccctgtcgtcctctctgtccatttcaaagcttgttttcgccaccacaggaagggaaagatcccgcggaggcatcctgcttcttgggttcctggtgtgggaccagcggtctcgtggctccatgtctctgcttctgcccctccggtcccagtcccggtcaccactgaaagaatggactgagtgaggtggtgaggactctcttctgttccgggtcatgtcgtcgtcgctggtcacgtcactgttgttgtcgtcttctggttggtacatctccttgtaattctccagcagagtgacgagcttctcacagttctccggcttttttgctcgcacccaaggcttgagcttttcagggatgatggtcaggtactgctcaaggaccaagagctcgatgatctcctccttggtgcgggtctccggctgcaaccaatcgaggcagaggtttcggagtttgatcagggtcttccgaggcccaacaaattccacatagattaggttccgaaacctctgatgaaaaaactcagagtcagttggaccttctcctatgatgacatccggctccttagtcaagtcactgtctagctcatacagatttggggcccaggacttcttaggtttggtggcagacaagtgctttggaggcagcatttctctaagtaaaattttcactggaggaaccaaacatgagtcaacaggaaagacgcggcagcctgtgaccgtcagtactcagggacctgtctgggaacaggatcctttctggaacttcagaccaagcagctatccacaggaacagagtcaaaacacaggtatctggacccagccacctagcgtttggacctagtccctcttcctctcgccagtcgtctccaagaaggacggaagatcaagaaggcaaagctcacctcagtgctgcgcagcctcgggcacgaacagccgcctagcgcaccctcatggcgcccggcgcccggcggcgccaccagcccagggtggacatctcccgcgcctcccaaacctctcctcccgcagctgcccagacttctgc

SEQ ID NO: 16565 - RNA, 1851 nt, Homo sapiens
  source 1..1851: mol_type = other RNA
gtgggctgggctgggctgggcctaaaggtttccccgcgctcacgttcacgttcacgttcatgttcacgctcattatctttgtcatccccaaagtggattttctggtgctcaatcagggcagaactatgaaggaaggtttccttacacaccctgcactcgtagaatttgtctttgccatatattttctgaagctcactaaaggtggggctaggcatgaaggcttcctcacattcctgattcttacattccacaagataacctctagcatgaatcttccgatgttcagccaaggcggcactcttattgaaggtctctccacagtccttacattcaaaacgtttccctccaacctgacttttctgaacttcactgacagccacactgtggataaaggactcaccatactcatagaggttctctctagtatgcatgatctggtgctcaacaaattctgagatgacactgaacgacctcccacactcatcacatacatatggcattgccccaaaatcaattggctgtgactcggtaaaggagggggagctgaggctgctcaggctgctcacgctcatggcttttctcatctcactaccacattcaaagggcttcttcctgggacagcctttttgatcgtgaatcgagcccttcccatctgtgtcaaaatgatagcgcctctttctttcaagaactctctttctggaaacaagggttgaattaaacctaaagcctcccctaaatgcattcccttcataaacccgctgctggatcactgactccctcttgttcaatgaaatgtccttccagttatcatctgacattctggggaatctctgtgaccggtcgcttgactcccttgctcttcccgatttggaactgcgtgacacatccttgatgaatttttccattatcactccgtgggaagattcatcttcacaaatcccccgccggtgggttgattttttggcttcaggcatagtttttagaccgagggagagcagcttcctgtagttttccatgttgtcctggattgtgttgtgaggtttcctgtcctcagcgaggtccaccacattttggtatgattcagcatcctgagatcgggactcataagccctggagtccctgtcgtcctctctgtccatttcaaagcttgttttcgccaccacaggaagggaaagatcccgcggaggcatcctgcttcttgggttcctggtgtgggaccagcggtctcgtggctccatgtctctgcttctgcccctccggtcccagtcccggtcaccactgaaagaatggactgagtgaggtggtgaggactctcttctgttccgggtcatgtcgtcgtcgctggtcacgtcactgttgttgtcgtcttctggttggtacatctccttgtaattctccagcagagtgacgagcttctcacagttctccggcttttttgctcgcacccaaggcttgagcttttcagggatgatggtcaggtactgctcaaggaccaagagctcgatgatctcctccttggtgcgggtctccggctgcaaccaatcgaggcagaggtttcggagtttgatcagggtcttccgaggcccaacaaattccacatagattaggttccgaaacctctggacccagccacctagcgtttggacctagtccctcttcctctcgccagtcgtctccaagaaggacggaagatcaagaaggcaaagctcacctcagtgctgcgcagcctcgggcacgaacagccgcctagcgcaccctcatggcgcccggcgcccggcggcgccaccagcccagggtggacatctcccgcgcctcccaaacctctcctcccgcagctgcccagacttctgc

SEQ ID NO: 16566 - RNA, 1764 nt, Homo sapiens
  source 1..1764: mol_type = other RNA
gtgggctgggctgggctgggcctaaaggtttccccgcgctcacgttcacgttcacgttcatgttcacgctcattatctttgtcatccccaaagtggattttctggtgctcaatcagggcagaactatgaaggaaggtttccttacacaccctgcactcgtagaatttgtctttgccatatattttctgaagctcactaaaggtggggctaggcatgaaggcttcctcacattcctgattcttacattccacaagataacctctagcatgaatcttccgatgttcagccaaggcggcactcttattgaaggtctctccacagtccttacattcaaaacgtttccctccaacctgacttttctgaacttcactgacagccacactgtggataaaggactcaccatactcatagaggttctctctagtatgcatgatctggtgctcaacaaattctgagatgacactgaacgacctcccacactcatcacatacatatggcattgccccaaaatcaattggctgtgactcggtaaaggagggggagctgaggctgctcaggctgctcacgctcatggcttttctcatctcactaccacattcaaagggcttcttcctgggacagcctttttgatcgtgaatcgagcccttcccatctgtgtcaaaatgatagcgcctctttctttcaagaactctctttctggaaacaagggttgaattaaacctaaagcctcccctaaatgcattcccttcataaacccgctgctggatcactgactccctcttgttcaatgaaatgtccttccagttatcatctgacattctggggaatctctgtgaccggtcgcttgactcccttgctcttcccgatttggaactgcgtgacacatccttgatgaatttttccattatcactccgtgggaagattcatcttcacaaatcccccgccggtgggttgattttttggcttcaggcatagtttttagaccgagggagagcagcttcctgtagttttccatgttgtcctggattgtgttgtgaggtttcctgtcctcagcgaggtccaccacattttggtatgattcagcatcctgagatcgggactcataagccctggagtccctgtcgtcctctctgtccatttcaaagcttgttttcgccaccacaggaagggaaagatcccgcggaggcatcctgcttcttgggttcctggtgtgggaccagcggtctcgtggctccatgtctctgcttctgcccctccggtcccagtcccggtcaccactgaaagaatggactgagtgaggtggtgaggactctcttctgttccgggtcatgtcgtcgtcgctggtcacgtcactgttgttgtcgtcttctggttggtacatctccttgtaattctccagcagagtgacgagcttctcacagttctccggcttttttgctcgcacccaaggcttgagcttttcagggatgatggtcaggtactgctcaaggaccaagagctcgatgatctcctccttggtgcgggtctccggctggacccagccacctagcgtttggacctagtccctcttcctctcgccagtcgtctccaagaaggacggaagatcaagaaggcaaagctcacctcagtgctgcgcagcctcgggcacgaacagccgcctagcgcaccctcatggcgcccggcgcccggcggcgccaccagcccagggtggacatctcccgcgcctcccaaacctctcctcccgcagctgcccagacttctgc

SEQ ID NO: 16567 - RNA, 1971 nt, Homo sapiens
  source 1..1971: mol_type = other RNA
gtgggctgggctgggctgggcctaaaggtttccccgcgctcacgttcacgttcacgttcatgttcacgctcattatctttgtcatccccaaagtggattttctggtgctcaatcagggcagaactatgaaggaaggtttccttacacaccctgcactcgtagaatttgtctttgccatatattttctgaagctcactaaaggtggggctaggcatgaaggcttcctcacattcctgattcttacattccacaagataacctctagcatgaatcttccgatgttcagccaaggcggcactcttattgaaggtctctccacagtccttacattcaaaacgtttccctccaacctgacttttctgaacttcactgacagccacactgtggataaaggactcaccatactcatagaggttctctctagtatgcatgatctggtgctcaacaaattctgagatgacactgaacgacctcccacactcatcacatacatatggcattgccccaaaatcaattggctgtgactcggtaaaggagggggagctgaggctgctcaggctgctcacgctcatggcttttctcatctcactaccacattcaaagggcttcttcctgggacagcctttttgatcgtgaatcgagcccttcccatctgtgtcaaaatgatagcgcctctttctttcaagaactctctttctggaaacaagggttgaattaaacctaaagcctcccctaaatgcattcccttcataaacccgctgctggatcactgactccctcttgttcaatgaaatgtccttccagttatcatctgacattctggggaatctctgtgaccggtcgcttgactcccttgctcttcccgatttggaactgcgtgacacatccttgatgaatttttccattatcactccgtgggaagattcatcttcacaaatcccccgccggtgggttgattttttggcttcaggcatagtttttagaccgagggagagcagcttcctgtagttttccatgttgtcctggattgtgttgtgaggtttcctgtcctcagcgaggtccaccacattttggtatgattcagcatcctgagatcgggactcataagccctggagtccctgtcgtcctctctgtccatttcaaagcttgttttcgccaccacaggaagggaaagatcccgcggaggcatcctgcttcttgggttcctggtgtgggaccagcggtctcgtggctccatgtctctgcttctgcccctccggtcccagtcccggtcaccactgaaagaatggactgagtgaggtggtgaggactctcttctgttccgggtcatgtcgtcgtcgctggtcacgtcactgttgttgtcgtcttctggttggtacatctccttgtaattctccagcagagtgacgagcttctcacagttctccggcttttttgctcgcacccaaggcttgagcttttcagggatgatggtcaggtactgctcaaggaccaagagctcgatgatctcctccttggtgcgggtctccggctgtctgggaacaggatcctttctggaacttcagaccaagcagctatccacaggaacagagtcaaaacacaggtatctcattaaaagggggctggaattgagaactttaaagtcaggaaccgaggaggttactctcttcgtctcccagggacagcgtggtgtgtggtctcgtctctcttcttgtttgctccattctcctgcctctctctggacccagccacctagcgtttggacctagtccctcttcctctcgccagtcgtctccaagaaggacggaagatcaagaaggcaaagctcacctcagtgctgcgcagcctcgggcacgaacagccgcctagcgcaccctcatggcgcccggcgcccggcggcgccaccagcccagggtggacatctcccgcgcctcccaaacctctcctcccgcagctgcccagacttctgc

SEQ ID NO: 16568 - RNA, 1840 nt, Homo sapiens
  source 1..1840: mol_type = other RNA
gtgggctgggctgggctgggcctaaaggtttccccgcgctcacgttcacgttcacgttcatgttcacgctcattatctttgtcatccccaaagtggattttctggtgctcaatcagggcagaactatgaaggaaggtttccttacacaccctgcactcgtagaatttgtctttgccatatattttctgaagctcactaaaggtggggctaggcatgaaggcttcctcacattcctgattcttacattccacaagataacctctagcatgaatcttccgatgttcagccaaggcggcactcttattgaaggtctctccacagtccttacattcaaaacgtttccctccaacctgacttttctgaacttcactgacagccacactgtggataaaggactcaccatactcatagaggttctctctagtatgcatgatctggtgctcaacaaattctgagatgacactgaacgacctcccacactcatcacatacatatggcattgccccaaaatcaattggctgtgactcggtaaaggagggggagctgaggctgctcaggctgctcacgctcatggcttttctcatctcactaccacattcaaagggcttcttcctgggacagcctttttgatcgtgaatcgagcccttcccatctgtgtcaaaatgatagcgcctctttctttcaagaactctctttctggaaacaagggttgaattaaacctaaagcctcccctaaatgcattcccttcataaacccgctgctggatcactgactccctcttgttcaatgaaatgtccttccagttatcatctgacattctggggaatctctgtgaccggtcgcttgactcccttgctcttcccgatttggaactgcgtgacacatccttgatgaatttttccattatcactccgtgggaagattcatcttcacaaatcccccgccggtgggttgattttttggcttcaggcatagtttttagaccgagggagagcagcttcctgtagttttccatgttgtcctggattgtgttgtgaggtttcctgtcctcagcgaggtccaccacattttggtatgattcagcatcctgagatcgggactcataagccctggagtccctgtcgtcctctctgtccatttcaaagcttgttttcgccaccacaggaagggaaagatcccgcggaggcatcctgcttcttgggttcctggtgtgggaccagcggtctcgtggctccatgtctctgcttctgcccctccggtcccagtcccggtcaccactgaaagaatggactgagtgaggtggtgaggactctcttctgttccgggtcatgtcgtcgtcgctggtcacgtcactgttgttgtcgtcttctggttggtacatctccttgtaattctccagcagagtgacgagcttctcacagttctccggcttttttgctcgcacccaaggcttgagcttttcagggatgatggtcaggtactgctcaaggaccaagagctcgatgatctcctccttggtgcgggtctccggctgtctgggaacaggatcctttctggaacttcagaccaagcagctatccacaggaacagagtcaaaacacaggtatctggacccagccacctagcgtttggacctagtccctcttcctctcgccagtcgtctccaagaaggacggaagatcaagaaggcaaagctcacctcagtgctgcgcagcctcgggcacgaacagccgcctagcgcaccctcatggcgcccggcgcccggcggcgccaccagcccagggtggacatctcccgcgcctcccaaacctctcctcccgcagctgcccagacttctgc

SEQ ID NO: 16569 - RNA, 1835 nt, Homo sapiens
  source 1..1835: mol_type = other RNA
gtgggctgggctgggctgggcctaaaggtttccccgcgctcacgttcacgttcacgttcatgttcacgctcattatctttgtcatccccaaagtggattttctggtgctcaatcagggcagaactatgaaggaaggtttccttacacaccctgcactcgtagaatttgtctttgccatatattttctgaagctcactaaaggtggggctaggcatgaaggcttcctcacattcctgattcttacattccacaagataacctctagcatgaatcttccgatgttcagccaaggcggcactcttattgaaggtctctccacagtccttacattcaaaacgtttccctccaacctgacttttctgaacttcactgacagccacactgtggataaaggactcaccatactcatagaggttctctctagtatgcatgatctggtgctcaacaaattctgagatgacactgaacgacctcccacactcatcacatacatatggcattgccccaaaatcaattggctgtgactcggtaaaggagggggagctgaggctgctcaggctgctcacgctcatggcttttctcatctcactaccacattcaaagggcttcttcctgggacagcctttttgatcgtgaatcgagcccttcccatctgtgtcaaaatgatagcgcctctttctttcaagaactctctttctggaaacaagggttgaattaaacctaaagcctcccctaaatgcattcccttcataaacccgctgctggatcactgactccctcttgttcaatgaaatgtccttccagttatcatctgacattctggggaatctctgtgaccggtcgcttgactcccttgctcttcccgatttggaactgcgtgacacatccttgatgaatttttccattatcactccgtgggaagattcatcttcacaaatcccccgccggtgggttgattttttggcttcaggcatagtttttagaccgagggagagcagcttcctgtagttttccatgttgtcctggattgtgttgtgaggtttcctgtcctcagcgaggtccaccacattttggtatgattcagcatcctgagatcgggactcataagccctggagtccctgtcgtcctctctgtccatttcaaagcttgttttcgccaccacaggaagggaaagatcccgcggaggcatcctgcttcttgggttcctggtgtgggaccagcggtctcgtggctccatgtctctgcttctgcccctccggtcccagtcccggtcaccactgaaagaatggactgagtgaggtggtgaggactctcttctgttccgggtcatgtcgtcgtcgctggtcacgtcactgttgttgtcgtcttctggttggtacatctccttgtaattctccagcagagtgacgagcttctcacagttctccggcttttttgctcgcacccaaggcttgagcttttcagggatgatggtcaggtactgctcaaggaccaagagctcgatgatctcctccttggtgcgggtctccggctgtctgggaacaggatcctttctggaacttcagaccaagcagctatccacaggaacagagtcaaaacacaggtatctggacccagccacctagcgtttggacctagtccctcttcctctcgccagtcgtctccaagaaggacggaagatcaagaaggcaaagctcagtgctgcgcagcctcgggcacgaacagccgcctagcgcaccctcatggcgcccggcgcccggcggcgccaccagcccagggtggacatctcccgcgcctcccaaacctctcctcccgcagctgcccagacttctgc

SEQ ID NO: 16570 - RNA, 2165 nt, Homo sapiens
  source 1..2165: mol_type = other RNA
gtgggctgggctgggctgggcctaaaggtttccccgcgctcacgttcacgttcacgttcatgttcacgctcattatctttgtcatccccaaagtggattttctggtgctcaatcagggcagaactatgaaggaaggtttccttacacaccctgcactcgtagaatttgtctttgccatatattttctgaagctcactaaaggtggggctaggcatgaaggcttcctcacattcctgattcttacattccacaagataacctctagcatgaatcttccgatgttcagccaaggcggcactcttattgaaggtctctccacagtccttacattcaaaacgtttccctccaacctgacttttctgaacttcactgacagccacactgtggataaaggactcaccatactcatagaggttctctctagtatgcatgatctggtgctcaacaaattctgagatgacactgaacgacctcccacactcatcacatacatatggcattgccccaaaatcaattggctgtgactcggtaaaggagggggagctgaggctgctcaggctgctcacgctcatggcttttctcatctcactaccacattcaaagggcttcttcctgggacagcctttttgatcgtgaatcgagcccttcccatctgtgtcaaaatgatagcgcctctttctttcaagaactctctttctggaaacaagggttgaattaaacctaaagcctcccctaaatgcattcccttcataaacccgctgctggatcactgactccctcttgttcaatgaaatgtccttccagttatcatctgacattctggggaatctctgtgaccggtcgcttgactcccttgctcttcccgatttggaactgcgtgacacatccttgatgaatttttccattatcactccgtgggaagattcatcttcacaaatcccccgccggtgggttgattttttggcttcaggcatagtttttagacctcgactggtgcttgggtaggcacttctcttggatcttgatgagtggccctgcgtcatgtgggagtggccatcgtcttcagcaagctgcacgagggagagcagcttcctgtagttttccatgttgtcctggattgtgttgtgaggtttcctgtcctcagcgaggtccaccacattttggtatgattcagcatcctgagatcgggactcataagccctggagtccctgtcgtcctctctgtccatttcaaagcttgttttcgccaccacaggaagggaaagatcccgcggaggcatcctgcttcttgggttcctggtgtgggaccagcggtctcgtggctccatgtctctgcttctgcccctccggtcccagtcccggtcactgaaagaatggactgagtgaggtggtgaggactctcttctgttccgggtcatgtcgtcgtcgctggtcacgtcactgttgttgtcgtcttctggttggtacatctccttgtaattctccagcagagtgacgagcttctcacagttctccggcttttttgctcgcacccaaggcttgagcttttcagggatgatggtcaggtactgctcaaggaccaagagctcgatgatctcctccttggtgcgggtctccggctgcaaccaatcgaggcagaggtttcggagtttgatcagggtcttccgaggcccaacaaattccacatagattaggttccgaaacctctgatgaaaaaactcagagtcagttggaccttctcctatgatgacatccggctccttagtcaagtcactgtctagctcatacagatttggggcccaggacttcttaggtttggtggcagacaagtgctttggaggcagcatttctctaagtaaaattttcactggaggaaccaaacatgagtcaacaggaaagacgcggcagcctgtgaccgtcagtactcagggacctggacccagccacctagcgtttggacctagtccctcttcctctcgccagtcgtctccaagaaggacggaagatcaagaaggcaaagctcacctcagtgctgcgcagcctcgggcacgaacagccgcctagcgcaccctcatggcgcccggcgcccggcggcgccaccagcccagggtggacatctcccgcgcctcccaaacctctcctcccgcagctgcccagacttctgc

SEQ ID NO: 16571 - RNA, 2241 nt, Homo sapiens
  source 1..2241: mol_type = other RNA
gtgggctgggctgggctgggcctaaaggtttccccgcgctcacgttcacgttcacgttcatgttcacgctcattatctttgtcatccccaaagtggattttctggtgctcaatcagggcagaactatgaaggaaggtttccttacacaccctgcactcgtagaatttgtctttgccatatattttctgaagctcactaaaggtggggctaggcatgaaggcttcctcacattcctgattcttacattccacaagataacctctagcatgaatcttccgatgttcagccaaggcggcactcttattgaaggtctctccacagtccttacattcaaaacgtttccctccaacctgacttttctgaacttcactgacagccacactgtggataaaggactcaccatactcatagaggttctctctagtatgcatgatctggtgctcaacaaattctgagatgacactgaacgacctcccacactcatcacatacatatggcattgccccaaaatcaattggctgtgactcggtaaaggagggggagctgaggctgctcaggctgctcacgctcatggcttttctcatctcactaccacattcaaagggcttcttcctgggacagcctttttgatcgtgaatcgagcccttcccatctgtgtcaaaatgatagcgcctctttctttcaagaactctctttctggaaacaagggttgaattaaacctaaagcctcccctaaatgcattcccttcataaacccgctgctggatcactgactccctcttgttcaatgaaatgtccttccagttatcatctgacattctggggaatctctgtgaccggtcgcttgactcccttgctcttcccgatttggaactgcgtgacacatccttgatgaatttttccattatcactccgtgggaagattcatcttcacaaatcccccgccggtgggttgattttttggcttcaggcatagtttttagacctcgactggtgcttgggtaggcacttctcttggatcttgatgagtggccctgcgtcatgtgggagtggccatcgtcttcagcaagctgcacgagggagagcagcttcctgtagttttccatgttgtcctggattgtgttgtgaggtttcctgtcctcagcgaggtccaccacattttggtatgattcagcatcctgagatcgggactcataagccctggagtccctgtcgtcctctctgtccatttcaaagcttgttttcgccaccacaggaagggaaagatcccgcggaggcatcctgcttcttgggttcctggtgtgggaccagcggtctcgtggctccatgtctctgcttctgcccctccggtcccagtcccggtcactgaaagaatggactgagtgaggtggtgaggactctcttctgttccgggtcatgtcgtcgtcgctggtcacgtcactgttgttgtcgtcttctggttggtacatctccttgtaattctccagcagagtgacgagcttctcacagttctccggcttttttgctcgcacccaaggcttgagcttttcagggatgatggtcaggtactgctcaaggaccaagagctcgatgatctcctccttggtgcgggtctccggctgcaaccaatcgaggcagaggtttcggagtttgatcagggtcttccgaggcccaacaaattccacatagattaggttccgaaacctctgatgaaaaaactcagagtcagttggaccttctcctatgatgacatccggctccttagtcaagtcactgtctagctcatacagatttggggcccaggacttcttaggtttggtggcagacaagtgctttggaggcagcatttctctaagtaaaattttcactggaggaaccaaacatgagtcaacaggaaagacgcggcagcctgtgaccgtcagtactcagggacctgtctgggaacaggatcctttctggaacttcagaccaagcagctatccacaggaacagagtcaaaacacaggtatctggacccagccacctagcgtttggacctagtccctcttcctctcgccagtcgtctccaagaaggacggaagatcaagaaggcaaagctcacctcagtgctgcgcagcctcgggcacgaacagccgcctagcgcaccctcatggcgcccggcgcccggcggcgccaccagcccagggtggacatctcccgcgcctcccaaacctctcctcccgcagctgcccagacttctgc

SEQ ID NO: 16572 - RNA, 1851 nt, Homo sapiens
  source 1..1851: mol_type = other RNA
gtgggctgggctgggctgggcctaaaggtttccccgcgctcacgttcacgttcacgttcatgttcacgctcattatctttgtcatccccaaagtggattttctggtgctcaatcagggcagaactatgaaggaaggtttccttacacaccctgcactcgtagaatttgtctttgccatatattttctgaagctcactaaaggtggggctaggcatgaaggcttcctcacattcctgattcttacattccacaagataacctctagcatgaatcttccgatgttcagccaaggcggcactcttattgaaggtctctccacagtccttacattcaaaacgtttccctccaacctgacttttctgaacttcactgacagccacactgtggataaaggactcaccatactcatagaggttctctctagtatgcatgatctggtgctcaacaaattctgagatgacactgaacgacctcccacactcatcacatacatatggcattgccccaaaatcaattggctgtgactcggtaaaggagggggagctgaggctgctcaggctgctcacgctcatggcttttctcatctcactaccacattcaaagggcttcttcctgggacagcctttttgatcgtgaatcgagcccttcccatctgtgtcaaaatgatagcgcctctttctttcaagaactctctttctggaaacaagggttgaattaaacctaaagcctcccctaaatgcattcccttcataaacccgctgctggatcactgactccctcttgttcaatgaaatgtccttccagttatcatctgacattctggggaatctctgtgaccggtcgcttgactcccttgctcttcccgatttggaactgcgtgacacatccttgatgaatttttccattatcactccgtgggaagattcatcttcacaaatcccccgccggtgggttgattttttggcttcaggcatagtttttagacctcgactggtgcttgggtaggcacttctcttggatcttgatgagtggccctgcgtcatgtgggagtggccatcgtcttcagcaagctgcacgagggagagcagcttcctgtagttttccatgttgtcctggattgtgttgtgaggtttcctgtcctcagcgaggtccaccacattttggtatgattcagcatcctgagatcgggactcataagccctggagtccctgtcgtcctctctgtccatttcaaagcttgttttcgccaccacaggaagggaaagatcccgcggaggcatcctgcttcttgggttcctggtgtgggaccagcggtctcgtggctccatgtctctgcttctgcccctccggtcccagtcccggtcactgaaagaatggactgagtgaggtggtgaggactctcttctgttccgggtcatgtcgtcgtcgctggtcacgtcactgttgttgtcgtcttctggttggtacatctccttgtaattctccagcagagtgacgagcttctcacagttctccggcttttttgctcgcacccaaggcttgagcttttcagggatgatggtcaggtactgctcaaggaccaagagctcgatgatctcctccttggtgcgggtctccggctggacccagccacctagcgtttggacctagtccctcttcctctcgccagtcgtctccaagaaggacggaagatcaagaaggcaaagctcacctcagtgctgcgcagcctcgggcacgaacagccgcctagcgcaccctcatggcgcccggcgcccggcggcgccaccagcccagggtggacatctcccgcgcctcccaaacctctcctcccgcagctgcccagacttctgc

SEQ ID NO: 16573 - RNA, 1988 nt, Homo sapiens
  source 1..1988: mol_type = other RNA
gtgggctgggctgggctgggcctaaaggtttccccgcgctcacgttcacgttcacgttcatgttcacgctcattatctttgtcatccccaaagtggattttctggtgctcaatcagggcagaactatgaaggaaggtttccttacacaccctgcactcgtagaatttgtctttgccatatattttctgaagctcactaaaggtggggctaggcatgaaggcttcctcacattcctgattcttacattccacaagataacctctagcatgaatcttccgatgttcagccaaggcggcactcttattgaaggtctctccacagtccttacattcaaaacgtttccctccaacctgacttttctgaacttcactgacagccacactgtggataaaggactcaccatactcatagaggttctctctagtatgcatgatctggtgctcaacaaattctgagatgacactgaacgacctcccacactcatcacatacatatggcattgccccaaaatcaattggctgtgactcggtaaaggagggggagctgaggctgctcaggctgctcacgctcatggcttttctcatctcactaccacattcaaagggcttcttcctgggacagcctttttgatcgtgaatcgagcccttcccatctgtgtcaaaatgatagcgcctctttctttcaagaactctctttctggaaacaagggttgaattaaacctaaagcctcccctaaatgcattcccttcataaacccgctgctggatcactgactccctcttgttcaatgaaatgtccttccagttatcatctgacattctggggaatctctgtgaccggtcgcttgactcccttgctcttcccgatttggaactgcgtgacacatccttgatgaatttttccattatcactccgtgggaagattcatcttcacaaatcccccgccggtgggttgattttttggcttcaggcatagtttttagacctcgactggtgcttgggtaggcacttctcttggatcttgatgagtggccctgcgtcatgtgggagtggccatcgtcttcagcaagctgcactccgagggagagcagcttcctgtagttttccatgttgtcctggattgtgttgtgaggtttcctgtcctcagcgaggtccaccacattttggtatgattcagcatcctgagatcgggactcataagccctggagtccctgtcgtcctctctgtccatttcaaagcttgttttcgccaccacaggaagggaaagatcccgcggaggcatcctgcttcttgggttcctggtgtgggaccagcggtctcgtggctccatgtctctgcttctgcccctccggtcccagtcccggtcaccactgaaagaatggactgagtgaggtggtgaggactctcttctgttccgggtcatgtcgtcgtcgctggtcacgtcactgttgttgtcgtcttctggttggtacatctccttgtaattctccagcagagtgacgagcttctcacagttctccggcttttttgctcgcacccaaggcttgagcttttcagggatgatggtcaggtactgctcaaggaccaagagctcgatgatctcctccttggtgcgggtctccggctcattaaaagggggctggaattgagaactttaaagtcaggaaccgaggaggttactctcttcgtctcccagggacagcgtggtgtgtggtctcgtctctcttcttgtttgctccattctcctgcctctctctggacccagccacctagcgtttggacctagtccctcttcctctcgccagtcgtctccaagaaggacggaagatcaagaaggcaaagctcacctcagtgctgcgcagcctcgggcacgaacagccgcctagcgcaccctcatggcgcccggcgcccggcggcgccaccagcccagggtggacatctcccgcgcctcccaaacctctcctcccgcagctgcccagacttctgc

SEQ ID NO: 16574 - RNA, 2109 nt, Homo sapiens
  source 1..2109: mol_type = other RNA
gtgggctgggctgggctgggcctaaaggtttccccgcgctcacgttcacgttcacgttcatgttcacgctcattatctttgtcatccccaaagtggattttctggtgctcaatcagggcagaactatgaaggaaggtttccttacacaccctgcactcgtagaatttgtctttgccatatattttctgaagctcactaaaggtggggctaggcatgaaggcttcctcacattcctgattcttacattccacaagataacctctagcatgaatcttccgatgttcagccaaggcggcactcttattgaaggtctctccacagtccttacattcaaaacgtttccctccaacctgacttttctgaacttcactgacagccacactgtggataaaggactcaccatactcatagaggttctctctagtatgcatgatctggtgctcaacaaattctgagatgacactgaacgacctcccacactcatcacatacatatggcattgccccaaaatcaattggctgtgactcggtaaaggagggggagctgaggctgctcaggctgctcacgctcatggcttttctcatctcactaccacattcaaagggcttcttcctgggacagcctttttgatcgtgaatcgagcccttcccatctgtgtcaaaatgatagcgcctctttctttcaagaactctctttctggaaacaagggttgaattaaacctaaagcctcccctaaatgcattcccttcataaacccgctgctggatcactgactccctcttgttcaatgaaatgtccttccagttatcatctgacattctggggaatctctgtgaccggtcgcttgactcccttgctcttcccgatttggaactgcgtgacacatccttgatgaatttttccattatcactccgtgggaagattcatcttcacaaatcccccgccggtgggttgattttttggcttcaggcatagtttttagacctcgactggtgcttgggtaggcacttctcttggatcttgatgagtggccctgcgtcatgtgggagtggccatcgtcttcagcaagctgcactccgagggagagcagcttcctgtagttttccatgttgtcctggattgtgttgtgaggtttcctgtcctcagcgaggtccaccacattttggtatgattcagcatcctgagatcgggactcataagccctggagtccctgtcgtcctctctgtccatttcaaagcttgttttcgccaccacaggaagggaaagatcccgcggaggcatcctgcttcttgggttcctggtgtgggaccagcggtctcgtggctccatgtctctgcttctgcccctccggtcccagtcccggtcaccactgaaagaatggactgagtgaggtggtgaggactctcttctgttccgggtcatgtcgtcgtcgctggtcacgtcactgttgttgtcgtcttctggttggtacatctccttgtaattctccagcagagtgacgagcttctcacagttctccggcttttttgctcgcacccaaggcttgagcttttcagggatgatggtcaggtactgctcaaggaccaagagctcgatgatctcctccttggtgcgggtctccggctcattaaaagggggctggaattgagaactttaaagtcaggaaccgaggaggttactctcttcgtctcccagggacagcgtggtgtgtggtctcgtctctcttcttgtttgctccattctcctgcctctctctttccaggtgggatgactcaggaggtctgtggttccccaggaaagaagcattcctacaatcactccaggagctgttctttgagaaccactgctctaaggtatccagtctggtccaatcacctggacccagccacctagcgtttggacctagtccctcttcctctcgccagtcgtctccaagaaggacggaagatcaagaaggcaaagctcacctcagtgctgcgcagcctcgggcacgaacagccgcctagcgcaccctcatggcgcccggcgcccggcggcgccaccagcccagggtggacatctcccgcgcctcccaaacctctcctcccgcagctgcccagacttctgc

SEQ ID NO: 16575 - RNA, 2166 nt, Homo sapiens
  source 1..2166: mol_type = other RNA
gtgggctgggctgggctgggcctaaaggtttccccgcgctcacgttcacgttcacgttcatgttcacgctcattatctttgtcatccccaaagtggattttctggtgctcaatcagggcagaactatgaaggaaggtttccttacacaccctgcactcgtagaatttgtctttgccatatattttctgaagctcactaaaggtggggctaggcatgaaggcttcctcacattcctgattcttacattccacaagataacctctagcatgaatcttccgatgttcagccaaggcggcactcttattgaaggtctctccacagtccttacattcaaaacgtttccctccaacctgacttttctgaacttcactgacagccacactgtggataaaggactcaccatactcatagaggttctctctagtatgcatgatctggtgctcaacaaattctgagatgacactgaacgacctcccacactcatcacatacatatggcattgccccaaaatcaattggctgtgactcggtaaaggagggggagctgaggctgctcaggctgctcacgctcatggcttttctcatctcactaccacattcaaagggcttcttcctgggacagcctttttgatcgtgaatcgagcccttcccatctgtgtcaaaatgatagcgcctctttctttcaagaactctctttctggaaacaagggttgaattaaacctaaagcctcccctaaatgcattcccttcataaacccgctgctggatcactgactccctcttgttcaatgaaatgtccttccagttatcatctgacattctggggaatctctgtgaccggtcgcttgactcccttgctcttcccgatttggaactgcgtgacacatccttgatgaatttttccattatcactccgtgggaagattcatcttcacaaatcccccgccggtgggttgattttttggcttcaggcatagtttttagacctcgactggtgcttgggtaggcacttctcttggatcttgatgagtggccctgcgtcatgtgggagtggccatcgtcttcagcaagctgcactccgagggagagcagcttcctgtagttttccatgttgtcctggattgtgttgtgaggtttcctgtcctcagcgaggtccaccacattttggtatgattcagcatcctgagatcgggactcataagccctggagtccctgtcgtcctctctgtccatttcaaagcttgttttcgccaccacaggaagggaaagatcccgcggaggcatcctgcttcttgggttcctggtgtgggaccagcggtctcgtggctccatgtctctgcttctgcccctccggtcccagtcccggtcaccactgaaagaatggactgagtgaggtggtgaggactctcttctgttccgggtcatgtcgtcgtcgctggtcacgtcactgttgttgtcgtcttctggttggtacatctccttgtaattctccagcagagtgacgagcttctcacagttctccggcttttttgctcgcacccaaggcttgagcttttcagggatgatggtcaggtactgctcaaggaccaagagctcgatgatctcctccttggtgcgggtctccggctgcaaccaatcgaggcagaggtttcggagtttgatcagggtcttccgaggcccaacaaattccacatagattaggttccgaaacctctgatgaaaaaactcagagtcagttggaccttctcctatgatgacatccggctccttagtcaagtcactgtctagctcatacagatttggggcccaggacttcttaggtttggtggcagacaagtgctttggaggcagcatttctctaagtaaaattttcactggaggaaccaaacatgagtcaacaggaaagacgcggcagcctgtgaccgtcagtactcagggacctggacccagccacctagcgtttggacctagtccctcttcctctcgccagtcgtctccaagaaggacggaagatcaagaaggcaaagctcagtgctgcgcagcctcgggcacgaacagccgcctagcgcaccctcatggcgcccggcgcccggcggcgccaccagcccagggtggacatctcccgcgcctcccaaacctctcctcccgcagctgcccagacttctgc

SEQ ID NO: 16576 - RNA, 2247 nt, Homo sapiens
  source 1..2247: mol_type = other RNA
gtgggctgggctgggctgggcctaaaggtttccccgcgctcacgttcacgttcacgttcatgttcacgctcattatctttgtcatccccaaagtggattttctggtgctcaatcagggcagaactatgaaggaaggtttccttacacaccctgcactcgtagaatttgtctttgccatatattttctgaagctcactaaaggtggggctaggcatgaaggcttcctcacattcctgattcttacattccacaagataacctctagcatgaatcttccgatgttcagccaaggcggcactcttattgaaggtctctccacagtccttacattcaaaacgtttccctccaacctgacttttctgaacttcactgacagccacactgtggataaaggactcaccatactcatagaggttctctctagtatgcatgatctggtgctcaacaaattctgagatgacactgaacgacctcccacactcatcacatacatatggcattgccccaaaatcaattggctgtgactcggtaaaggagggggagctgaggctgctcaggctgctcacgctcatggcttttctcatctcactaccacattcaaagggcttcttcctgggacagcctttttgatcgtgaatcgagcccttcccatctgtgtcaaaatgatagcgcctctttctttcaagaactctctttctggaaacaagggttgaattaaacctaaagcctcccctaaatgcattcccttcataaacccgctgctggatcactgactccctcttgttcaatgaaatgtccttccagttatcatctgacattctggggaatctctgtgaccggtcgcttgactcccttgctcttcccgatttggaactgcgtgacacatccttgatgaatttttccattatcactccgtgggaagattcatcttcacaaatcccccgccggtgggttgattttttggcttcaggcatagtttttagacctcgactggtgcttgggtaggcacttctcttggatcttgatgagtggccctgcgtcatgtgggagtggccatcgtcttcagcaagctgcactccgagggagagcagcttcctgtagttttccatgttgtcctggattgtgttgtgaggtttcctgtcctcagcgaggtccaccacattttggtatgattcagcatcctgagatcgggactcataagccctggagtccctgtcgtcctctctgtccatttcaaagcttgttttcgccaccacaggaagggaaagatcccgcggaggcatcctgcttcttgggttcctggtgtgggaccagcggtctcgtggctccatgtctctgcttctgcccctccggtcccagtcccggtcaccactgaaagaatggactgagtgaggtggtgaggactctcttctgttccgggtcatgtcgtcgtcgctggtcacgtcactgttgttgtcgtcttctggttggtacatctccttgtaattctccagcagagtgacgagcttctcacagttctccggcttttttgctcgcacccaaggcttgagcttttcagggatgatggtcaggtactgctcaaggaccaagagctcgatgatctcctccttggtgcgggtctccggctgcaaccaatcgaggcagaggtttcggagtttgatcagggtcttccgaggcccaacaaattccacatagattaggttccgaaacctctgatgaaaaaactcagagtcagttggaccttctcctatgatgacatccggctccttagtcaagtcactgtctagctcatacagatttggggcccaggacttcttaggtttggtggcagacaagtgctttggaggcagcatttctctaagtaaaattttcactggaggaaccaaacatgagtcaacaggaaagacgcggcagcctgtgaccgtcagtactcagggacctgtctgggaacaggatcctttctggaacttcagaccaagcagctatccacaggaacagagtcaaaacacaggtatctggacccagccacctagcgtttggacctagtccctcttcctctcgccagtcgtctccaagaaggacggaagatcaagaaggcaaagctcacctcagtgctgcgcagcctcgggcacgaacagccgcctagcgcaccctcatggcgcccggcgcccggcggcgccaccagcccagggtggacatctcccgcgcctcccaaacctctcctcccgcagctgcccagacttctgc

SEQ ID NO: 16577 - RNA, 1939 nt, Homo sapiens
  source 1..1939: mol_type = other RNA
gtgggctgggctgggctgggcctaaaggtttccccgcgctcacgttcacgttcacgttcatgttcacgctcattatctttgtcatccccaaagtggattttctggtgctcaatcagggcagaactatgaaggaaggtttccttacacaccctgcactcgtagaatttgtctttgccatatattttctgaagctcactaaaggtggggctaggcatgaaggcttcctcacattcctgattcttacattccacaagataacctctagcatgaatcttccgatgttcagccaaggcggcactcttattgaaggtctctccacagtccttacattcaaaacgtttccctccaacctgacttttctgaacttcactgacagccacactgtggataaaggactcaccatactcatagaggttctctctagtatgcatgatctggtgctcaacaaattctgagatgacactgaacgacctcccacactcatcacatacatatggcattgccccaaaatcaattggctgtgactcggtaaaggagggggagctgaggctgctcaggctgctcacgctcatggcttttctcatctcactaccacattcaaagggcttcttcctgggacagcctttttgatcgtgaatcgagcccttcccatctgtgtcaaaatgatagcgcctctttctttcaagaactctctttctggaaacaagggttgaattaaacctaaagcctcccctaaatgcattcccttcataaacccgctgctggatcactgactccctcttgttcaatgaaatgtccttccagttatcatctgacattctggggaatctctgtgaccggtcgcttgactcccttgctcttcccgatttggaactgcgtgacacatccttgatgaatttttccattatcactccgtgggaagattcatcttcacaaatcccccgccggtgggttgattttttggcttcaggcatagtttttagacctcgactggtgcttgggtaggcacttctcttggatcttgatgagtggccctgcgtcatgtgggagtggccatcgtcttcagcaagctgcactccgagggagagcagcttcctgtagttttccatgttgtcctggattgtgttgtgaggtttcctgtcctcagcgaggtccaccacattttggtatgattcagcatcctgagatcgggactcataagccctggagtccctgtcgtcctctctgtccatttcaaagcttgttttcgccaccacaggaagggaaagatcccgcggaggcatcctgcttcttgggttcctggtgtgggaccagcggtctcgtggctccatgtctctgcttctgcccctccggtcccagtcccggtcaccactgaaagaatggactgagtgaggtggtgaggactctcttctgttccgggtcatgtcgtcgtcgctggtcacgtcactgttgttgtcgtcttctggttggtacatctccttgtaattctccagcagagtgacgagcttctcacagttctccggcttttttgctcgcacccaaggcttgagcttttcagggatgatggtcaggtactgctcaaggaccaagagctcgatgatctcctccttggtgcgggtctccggctgcaaccaatcgaggcagaggtttcggagtttgatcagggtcttccgaggcccaacaaattccacatagattaggttccgaaacctctggacccagccacctagcgtttggacctagtccctcttcctctcgccagtcgtctccaagaaggacggaagatcaagaaggcaaagctcagtgctgcgcagcctcgggcacgaacagccgcctagcgcaccctcatggcgcccggcgcccggcggcgccaccagcccagggtggacatctcccgcgcctcccaaacctctcctcccgcagctgcccagacttctgc

SEQ ID NO: 16578 - RNA, 2020 nt, Homo sapiens
  source 1..2020: mol_type = other RNA
gtgggctgggctgggctgggcctaaaggtttccccgcgctcacgttcacgttcacgttcatgttcacgctcattatctttgtcatccccaaagtggattttctggtgctcaatcagggcagaactatgaaggaaggtttccttacacaccctgcactcgtagaatttgtctttgccatatattttctgaagctcactaaaggtggggctaggcatgaaggcttcctcacattcctgattcttacattccacaagataacctctagcatgaatcttccgatgttcagccaaggcggcactcttattgaaggtctctccacagtccttacattcaaaacgtttccctccaacctgacttttctgaacttcactgacagccacactgtggataaaggactcaccatactcatagaggttctctctagtatgcatgatctggtgctcaacaaattctgagatgacactgaacgacctcccacactcatcacatacatatggcattgccccaaaatcaattggctgtgactcggtaaaggagggggagctgaggctgctcaggctgctcacgctcatggcttttctcatctcactaccacattcaaagggcttcttcctgggacagcctttttgatcgtgaatcgagcccttcccatctgtgtcaaaatgatagcgcctctttctttcaagaactctctttctggaaacaagggttgaattaaacctaaagcctcccctaaatgcattcccttcataaacccgctgctggatcactgactccctcttgttcaatgaaatgtccttccagttatcatctgacattctggggaatctctgtgaccggtcgcttgactcccttgctcttcccgatttggaactgcgtgacacatccttgatgaatttttccattatcactccgtgggaagattcatcttcacaaatcccccgccggtgggttgattttttggcttcaggcatagtttttagacctcgactggtgcttgggtaggcacttctcttggatcttgatgagtggccctgcgtcatgtgggagtggccatcgtcttcagcaagctgcactccgagggagagcagcttcctgtagttttccatgttgtcctggattgtgttgtgaggtttcctgtcctcagcgaggtccaccacattttggtatgattcagcatcctgagatcgggactcataagccctggagtccctgtcgtcctctctgtccatttcaaagcttgttttcgccaccacaggaagggaaagatcccgcggaggcatcctgcttcttgggttcctggtgtgggaccagcggtctcgtggctccatgtctctgcttctgcccctccggtcccagtcccggtcaccactgaaagaatggactgagtgaggtggtgaggactctcttctgttccgggtcatgtcgtcgtcgctggtcacgtcactgttgttgtcgtcttctggttggtacatctccttgtaattctccagcagagtgacgagcttctcacagttctccggcttttttgctcgcacccaaggcttgagcttttcagggatgatggtcaggtactgctcaaggaccaagagctcgatgatctcctccttggtgcgggtctccggctgcaaccaatcgaggcagaggtttcggagtttgatcagggtcttccgaggcccaacaaattccacatagattaggttccgaaacctctgtctgggaacaggatcctttctggaacttcagaccaagcagctatccacaggaacagagtcaaaacacaggtatctggacccagccacctagcgtttggacctagtccctcttcctctcgccagtcgtctccaagaaggacggaagatcaagaaggcaaagctcacctcagtgctgcgcagcctcgggcacgaacagccgcctagcgcaccctcatggcgcccggcgcccggcggcgccaccagcccagggtggacatctcccgcgcctcccaaacctctcctcccgcagctgcccagacttctgc

SEQ ID NO: 16579 - RNA, 2015 nt, Homo sapiens
  source 1..2015: mol_type = other RNA
gtgggctgggctgggctgggcctaaaggtttccccgcgctcacgttcacgttcacgttcatgttcacgctcattatctttgtcatccccaaagtggattttctggtgctcaatcagggcagaactatgaaggaaggtttccttacacaccctgcactcgtagaatttgtctttgccatatattttctgaagctcactaaaggtggggctaggcatgaaggcttcctcacattcctgattcttacattccacaagataacctctagcatgaatcttccgatgttcagccaaggcggcactcttattgaaggtctctccacagtccttacattcaaaacgtttccctccaacctgacttttctgaacttcactgacagccacactgtggataaaggactcaccatactcatagaggttctctctagtatgcatgatctggtgctcaacaaattctgagatgacactgaacgacctcccacactcatcacatacatatggcattgccccaaaatcaattggctgtgactcggtaaaggagggggagctgaggctgctcaggctgctcacgctcatggcttttctcatctcactaccacattcaaagggcttcttcctgggacagcctttttgatcgtgaatcgagcccttcccatctgtgtcaaaatgatagcgcctctttctttcaagaactctctttctggaaacaagggttgaattaaacctaaagcctcccctaaatgcattcccttcataaacccgctgctggatcactgactccctcttgttcaatgaaatgtccttccagttatcatctgacattctggggaatctctgtgaccggtcgcttgactcccttgctcttcccgatttggaactgcgtgacacatccttgatgaatttttccattatcactccgtgggaagattcatcttcacaaatcccccgccggtgggttgattttttggcttcaggcatagtttttagacctcgactggtgcttgggtaggcacttctcttggatcttgatgagtggccctgcgtcatgtgggagtggccatcgtcttcagcaagctgcactccgagggagagcagcttcctgtagttttccatgttgtcctggattgtgttgtgaggtttcctgtcctcagcgaggtccaccacattttggtatgattcagcatcctgagatcgggactcataagccctggagtccctgtcgtcctctctgtccatttcaaagcttgttttcgccaccacaggaagggaaagatcccgcggaggcatcctgcttcttgggttcctggtgtgggaccagcggtctcgtggctccatgtctctgcttctgcccctccggtcccagtcccggtcaccactgaaagaatggactgagtgaggtggtgaggactctcttctgttccgggtcatgtcgtcgtcgctggtcacgtcactgttgttgtcgtcttctggttggtacatctccttgtaattctccagcagagtgacgagcttctcacagttctccggcttttttgctcgcacccaaggcttgagcttttcagggatgatggtcaggtactgctcaaggaccaagagctcgatgatctcctccttggtgcgggtctccggctgcaaccaatcgaggcagaggtttcggagtttgatcagggtcttccgaggcccaacaaattccacatagattaggttccgaaacctctgtctgggaacaggatcctttctggaacttcagaccaagcagctatccacaggaacagagtcaaaacacaggtatctggacccagccacctagcgtttggacctagtccctcttcctctcgccagtcgtctccaagaaggacggaagatcaagaaggcaaagctcagtgctgcgcagcctcgggcacgaacagccgcctagcgcaccctcatggcgcccggcgcccggcggcgccaccagcccagggtggacatctcccgcgcctcccaaacctctcctcccgcagctgcccagacttctgc

SEQ ID NO: 16580 - RNA, 2018 nt, Homo sapiens
  source 1..2018: mol_type = other RNA
gtgggctgggctgggctgggcctaaaggtttccccgcgctcacgttcacgttcacgttcatgttcacgctcattatctttgtcatccccaaagtggattttctggtgctcaatcagggcagaactatgaaggaaggtttccttacacaccctgcactcgtagaatttgtctttgccatatattttctgaagctcactaaaggtggggctaggcatgaaggcttcctcacattcctgattcttacattccacaagataacctctagcatgaatcttccgatgttcagccaaggcggcactcttattgaaggtctctccacagtccttacattcaaaacgtttccctccaacctgacttttctgaacttcactgacagccacactgtggataaaggactcaccatactcatagaggttctctctagtatgcatgatctggtgctcaacaaattctgagatgacactgaacgacctcccacactcatcacatacatatggcattgccccaaaatcaattggctgtgactcggtaaaggagggggagctgaggctgctcaggctgctcacgctcatggcttttctcatctcactaccacattcaaagggcttcttcctgggacagcctttttgatcgtgaatcgagcccttcccatctgtgtcaaaatgatagcgcctctttctttcaagaactctctttctggaaacaagggttgaattaaacctaaagcctcccctaaatgcattcccttcataaacccgctgctggatcactgactccctcttgttcaatgaaatgtccttccagttatcatctgacattctggggaatctctgtgaccggtcgcttgactcccttgctcttcccgatttggaactgcgtgacacatccttgatgaatttttccattatcactccgtgggaagattcatcttcacaaatcccccgccggtgggttgattttttggcttcaggcatagtttttagacctcgactggtgcttgggtaggcacttctcttggatcttgatgagtggccctgcgtcatgtgggagtggccatcgtcttcagcaagctgcactccgagggagagcagcttcctgtagttttccatgttgtcctggattgtgttgtgaggtttcctgtcctcagcgaggtccaccacattttggtatgattcagcatcctgagatcgggactcataagccctggagtccctgtcgtcctctctgtccatttcaaagcttgttttcgccaccacaggaagggaaagatcccgcggaggcatcctgcttcttgggttcctggtgtgggaccagcggtctcgtggctccatgtctctgcttctgcccctccggtcccagtcccggtcaccactgaaagaatggactgagtgaggtggtgaggactctcttctgttccgggtcatgtcgtcgtcgctggtcacgtcactgttgttgtcgtcttctggttggtacatctccttgtaattctccagcagagtgacgagcttctcacagttctccggcttttttgctcgcacccaaggcttgagcttttcagggatgatggtcaggtactgctcaaggaccaagagctcgatgatctcctccttggtgcgggtctccggctgcaaccaatcgaggcagaggtttcggagtttgatcagggtcttccgaggcccaacaaattccacatagattaggttccgaaacctgtctgggaacaggatcctttctggaacttcagaccaagcagctatccacaggaacagagtcaaaacacaggtatctggacccagccacctagcgtttggacctagtccctcttcctctcgccagtcgtctccaagaaggacggaagatcaagaaggcaaagctcacctcagtgctgcgcagcctcgggcacgaacagccgcctagcgcaccctcatggcgcccggcgcccggcggcgccaccagcccagggtggacatctcccgcgcctcccaaacctctcctcccgcagctgcccagacttctgc

SEQ ID NO: 16581 - RNA, 1857 nt, Homo sapiens
  source 1..1857: mol_type = other RNA
gtgggctgggctgggctgggcctaaaggtttccccgcgctcacgttcacgttcacgttcatgttcacgctcattatctttgtcatccccaaagtggattttctggtgctcaatcagggcagaactatgaaggaaggtttccttacacaccctgcactcgtagaatttgtctttgccatatattttctgaagctcactaaaggtggggctaggcatgaaggcttcctcacattcctgattcttacattccacaagataacctctagcatgaatcttccgatgttcagccaaggcggcactcttattgaaggtctctccacagtccttacattcaaaacgtttccctccaacctgacttttctgaacttcactgacagccacactgtggataaaggactcaccatactcatagaggttctctctagtatgcatgatctggtgctcaacaaattctgagatgacactgaacgacctcccacactcatcacatacatatggcattgccccaaaatcaattggctgtgactcggtaaaggagggggagctgaggctgctcaggctgctcacgctcatggcttttctcatctcactaccacattcaaagggcttcttcctgggacagcctttttgatcgtgaatcgagcccttcccatctgtgtcaaaatgatagcgcctctttctttcaagaactctctttctggaaacaagggttgaattaaacctaaagcctcccctaaatgcattcccttcataaacccgctgctggatcactgactccctcttgttcaatgaaatgtccttccagttatcatctgacattctggggaatctctgtgaccggtcgcttgactcccttgctcttcccgatttggaactgcgtgacacatccttgatgaatttttccattatcactccgtgggaagattcatcttcacaaatcccccgccggtgggttgattttttggcttcaggcatagtttttagacctcgactggtgcttgggtaggcacttctcttggatcttgatgagtggccctgcgtcatgtgggagtggccatcgtcttcagcaagctgcactccgagggagagcagcttcctgtagttttccatgttgtcctggattgtgttgtgaggtttcctgtcctcagcgaggtccaccacattttggtatgattcagcatcctgagatcgggactcataagccctggagtccctgtcgtcctctctgtccatttcaaagcttgttttcgccaccacaggaagggaaagatcccgcggaggcatcctgcttcttgggttcctggtgtgggaccagcggtctcgtggctccatgtctctgcttctgcccctccggtcccagtcccggtcaccactgaaagaatggactgagtgaggtggtgaggactctcttctgttccgggtcatgtcgtcgtcgctggtcacgtcactgttgttgtcgtcttctggttggtacatctccttgtaattctccagcagagtgacgagcttctcacagttctccggcttttttgctcgcacccaaggcttgagcttttcagggatgatggtcaggtactgctcaaggaccaagagctcgatgatctcctccttggtgcgggtctccggctggacccagccacctagcgtttggacctagtccctcttcctctcgccagtcgtctccaagaaggacggaagatcaagaaggcaaagctcacctcagtgctgcgcagcctcgggcacgaacagccgcctagcgcaccctcatggcgcccggcgcccggcggcgccaccagcccagggtggacatctcccgcgcctcccaaacctctcctcccgcagctgcccagacttctgc

SEQ ID NO: 16582 - RNA, 1852 nt, Homo sapiens
  source 1..1852: mol_type = other RNA
gtgggctgggctgggctgggcctaaaggtttccccgcgctcacgttcacgttcacgttcatgttcacgctcattatctttgtcatccccaaagtggattttctggtgctcaatcagggcagaactatgaaggaaggtttccttacacaccctgcactcgtagaatttgtctttgccatatattttctgaagctcactaaaggtggggctaggcatgaaggcttcctcacattcctgattcttacattccacaagataacctctagcatgaatcttccgatgttcagccaaggcggcactcttattgaaggtctctccacagtccttacattcaaaacgtttccctccaacctgacttttctgaacttcactgacagccacactgtggataaaggactcaccatactcatagaggttctctctagtatgcatgatctggtgctcaacaaattctgagatgacactgaacgacctcccacactcatcacatacatatggcattgccccaaaatcaattggctgtgactcggtaaaggagggggagctgaggctgctcaggctgctcacgctcatggcttttctcatctcactaccacattcaaagggcttcttcctgggacagcctttttgatcgtgaatcgagcccttcccatctgtgtcaaaatgatagcgcctctttctttcaagaactctctttctggaaacaagggttgaattaaacctaaagcctcccctaaatgcattcccttcataaacccgctgctggatcactgactccctcttgttcaatgaaatgtccttccagttatcatctgacattctggggaatctctgtgaccggtcgcttgactcccttgctcttcccgatttggaactgcgtgacacatccttgatgaatttttccattatcactccgtgggaagattcatcttcacaaatcccccgccggtgggttgattttttggcttcaggcatagtttttagacctcgactggtgcttgggtaggcacttctcttggatcttgatgagtggccctgcgtcatgtgggagtggccatcgtcttcagcaagctgcactccgagggagagcagcttcctgtagttttccatgttgtcctggattgtgttgtgaggtttcctgtcctcagcgaggtccaccacattttggtatgattcagcatcctgagatcgggactcataagccctggagtccctgtcgtcctctctgtccatttcaaagcttgttttcgccaccacaggaagggaaagatcccgcggaggcatcctgcttcttgggttcctggtgtgggaccagcggtctcgtggctccatgtctctgcttctgcccctccggtcccagtcccggtcaccactgaaagaatggactgagtgaggtggtgaggactctcttctgttccgggtcatgtcgtcgtcgctggtcacgtcactgttgttgtcgtcttctggttggtacatctccttgtaattctccagcagagtgacgagcttctcacagttctccggcttttttgctcgcacccaaggcttgagcttttcagggatgatggtcaggtactgctcaaggaccaagagctcgatgatctcctccttggtgcgggtctccggctggacccagccacctagcgtttggacctagtccctcttcctctcgccagtcgtctccaagaaggacggaagatcaagaaggcaaagctcagtgctgcgcagcctcgggcacgaacagccgcctagcgcaccctcatggcgcccggcgcccggcggcgccaccagcccagggtggacatctcccgcgcctcccaaacctctcctcccgcagctgcccagacttctgc

SEQ ID NO: 16583 - RNA, 1769 nt, Homo sapiens
  source 1..1769: mol_type = other RNA
gtgggctgggctgggctgggcctaaaggtttccccgcgctcacgttcacgttcacgttcatgttcacgctcattatctttgtcatccccaaagtggattttctggtgctcaatcagggcagaactatgaaggaaggtttccttacacaccctgcactcgtagaatttgtctttgccatatattttctgaagctcactaaaggtggggctaggcatgaaggcttcctcacattcctgattcttacattccacaagataacctctagcatgaatcttccgatgttcagccaaggcggcactcttattgaaggtctctccacagtccttacattcaaaacgtttccctccaacctgacttttctgaacttcactgacagccacactgtggataaaggactcaccatactcatagaggttctctctagtatgcatgatctggtgctcaacaaattctgagatgacactgaacgacctcccacactcatcacatacatatggcattgccccaaaatcaattggctgtgactcggtaaaggagggggagctgaggctgctcaggctgctcacgctcatggcttttctcatctcactaccacattcaaagggcttcttcctgggacagcctttttgatcgtgaatcgagcccttcccatctgtgtcaaaatgatagcgcctctttctttcaagaactctctttctggaaacaagggttgaattaaacctaaagcctcccctaaatgcattcccttcataaacccgctgctggatcactgactccctcttgttcaatgaaatgtccttccagttatcatctgacattctggggaatctctgtgaccggtcgcttgactcccttgctcttcccgatttggaactgcgtgacacatccttgatgaatttttccattatcactccgtgggaagattcatcttcacaaatcccccgccggtgggttgattttttggcttcaggcatagtttttagacctcgactggtgcttgggtaggcacttctcttggatcttgatgagtggccctgcgtcatgtgggagtggccatcgtcttcagcaagctgcactccgagggagagcagcttcctgtagttttccatgttgtcctggattgtgttgtgaggtttcctgtcctcagcgaggtccaccacattttggtatgattcagcatcctgagatcgggactcataagccctggagtccctgtcgtcctctctgtccatttcaaagcttgttttcgccaccacaggaagggaaagatcccgcggaggcatcctgcttcttgggttcctggtgtgggaccagcggtctcgtggctccatgtctctgcttctgcccctccggtcccagtcccggtcaccactgaaagaatggactgagtgaggtggtgaggactctcttctgttccgggtcatgtcgtcgtcgctggtcacgtcactgttgttgtcgtcttctggttggtacatctccttgtaattctccagcagagtgacgagcttctcacagttctccggcttttttgctcgcacccaaggcttgagcttttcagggatgatggtcaggtactgctcaaggaccaagagctcgatgatctcctccttggtgcgggtctccggctggacccagccacctagcgtttggacctagtccctcttcctctcgccagtcgtctccaagaaggacggaagatcaagaaggcaaagcttgaaatcccctcagccccctccaacagccctgctgtcactcaagatggcgcctgc

SEQ ID NO: 16584 - RNA, 2046 nt, Homo sapiens
  source 1..2046: mol_type = other RNA
gtgggctgggctgggctgggcctaaaggtttccccgcgctcacgttcacgttcacgttcatgttcacgctcattatctttgtcatccccaaagtggattttctggtgctcaatcagggcagaactatgaaggaaggtttccttacacaccctgcactcgtagaatttgtctttgccatatattttctgaagctcactaaaggtggggctaggcatgaaggcttcctcacattcctgattcttacattccacaagataacctctagcatgaatcttccgatgttcagccaaggcggcactcttattgaaggtctctccacagtccttacattcaaaacgtttccctccaacctgacttttctgaacttcactgacagccacactgtggataaaggactcaccatactcatagaggttctctctagtatgcatgatctggtgctcaacaaattctgagatgacactgaacgacctcccacactcatcacatacatatggcattgccccaaaatcaattggctgtgactcggtaaaggagggggagctgaggctgctcaggctgctcacgctcatggcttttctcatctcactaccacattcaaagggcttcttcctgggacagcctttttgatcgtgaatcgagcccttcccatctgtgtcaaaatgatagcgcctctttctttcaagaactctctttctggaaacaagggttgaattaaacctaaagcctcccctaaatgcattcccttcataaacccgctgctggatcactgactccctcttgttcaatgaaatgtccttccagttatcatctgacattctggggaatctctgtgaccggtcgcttgactcccttgctcttcccgatttggaactgcgtgacacatccttgatgaatttttccattatcactccgtgggaagattcatcttcacaaatcccccgccggtgggttgattttttggcttcaggcatagtttttagacctcgactggtgcttgggtaggcacttctcttggatcttgatgagtggccctgcgtcatgtgggagtggccatcgtcttcagcaagctgcactccgagggagagcagcttcctgtagttttccatgttgtcctggattgtgttgtgaggtttcctgtcctcagcgaggtccaccacattttggtatgattcagcatcctgagatcgggactcataagccctggagtccctgtcgtcctctctgtccatttcaaagcttgttttcgccaccacaggaagggaaagatcccgcggaggcatcctgcttcttgggttcctggtgtgggaccagcggtctcgtggctccatgtctctgcttctgcccctccggtcccagtcccggtcaccactgaaagaatggactgagtgaggtggtgaggactctcttctgttccgggtcatgtcgtcgtcgctggtcacgtcactgttgttgtcgtcttctggttggtacatctccttgtaattctccagcagagtgacgagcttctcacagttctccggcttttttgctcgcacccaaggcttgagcttttcagggatgatggtcaggtactgctcaaggaccaagagctcgatgatctcctccttggtgcgggtctccggctgtctgggaacaggatcctttctggaacttcagaccaagcagctatccacaggaacagagtcaaaacacaggtatcgtgttataaaaaccattccagagcacagaaaagagatggaggacttcctacaattaattttgtgaccacttgaatgcccatatgtatcttgtcacaaggtggatgccaacttctggacccagccacctagcgtttggacctagtccctcttcctctcgccagtcgtctccaagaaggacggaagatcaagaaggcaaagctcacctcagtgctgcgcagcctcgggcacgaacagccgcctagcgcaccctcatggcgcccggcgcccggcggcgccaccagcccagggtggacatctcccgcgcctcccaaacctctcctcccgcagctgcccagacttctgc

SEQ ID NO: 16585 - RNA, 2072 nt, Homo sapiens
  source 1..2072: mol_type = other RNA
gtgggctgggctgggctgggcctaaaggtttccccgcgctcacgttcacgttcacgttcatgttcacgctcattatctttgtcatccccaaagtggattttctggtgctcaatcagggcagaactatgaaggaaggtttccttacacaccctgcactcgtagaatttgtctttgccatatattttctgaagctcactaaaggtggggctaggcatgaaggcttcctcacattcctgattcttacattccacaagataacctctagcatgaatcttccgatgttcagccaaggcggcactcttattgaaggtctctccacagtccttacattcaaaacgtttccctccaacctgacttttctgaacttcactgacagccacactgtggataaaggactcaccatactcatagaggttctctctagtatgcatgatctggtgctcaacaaattctgagatgacactgaacgacctcccacactcatcacatacatatggcattgccccaaaatcaattggctgtgactcggtaaaggagggggagctgaggctgctcaggctgctcacgctcatggcttttctcatctcactaccacattcaaagggcttcttcctgggacagcctttttgatcgtgaatcgagcccttcccatctgtgtcaaaatgatagcgcctctttctttcaagaactctctttctggaaacaagggttgaattaaacctaaagcctcccctaaatgcattcccttcataaacccgctgctggatcactgactccctcttgttcaatgaaatgtccttccagttatcatctgacattctggggaatctctgtgaccggtcgcttgactcccttgctcttcccgatttggaactgcgtgacacatccttgatgaatttttccattatcactccgtgggaagattcatcttcacaaatcccccgccggtgggttgattttttggcttcaggcatagtttttagacctcgactggtgcttgggtaggcacttctcttggatcttgatgagtggccctgcgtcatgtgggagtggccatcgtcttcagcaagctgcactccgagggagagcagcttcctgtagttttccatgttgtcctggattgtgttgtgaggtttcctgtcctcagcgaggtccaccacattttggtatgattcagcatcctgagatcgggactcataagccctggagtccctgtcgtcctctctgtccatttcaaagcttgttttcgccaccacaggaagggaaagatcccgcggaggcatcctgcttcttgggttcctggtgtgggaccagcggtctcgtggctccatgtctctgcttctgcccctccggtcccagtcccggtcaccactgaaagaatggactgagtgaggtggtgaggactctcttctgttccgggtcatgtcgtcgtcgctggtcacgtcactgttgttgtcgtcttctggttggtacatctccttgtaattctccagcagagtgacgagcttctcacagttctccggcttttttgctcgcacccaaggcttgagcttttcagggatgatggtcaggtactgctcaaggaccaagagctcgatgatctcctccttggtgcgggtctccggctgtctgggaacaggatcctttctggaacttcagaccaagcagctatccacaggaacagagtcaaaacacaggtatctcaccctgactggggaagaccagatcccacgtgaccttctgtgacagcgagtctggccaatcaaaagcataactgctctgcccacttggcccccacttccccaggccagcttctccatggcaacagccacgcctaccactggacccagccacctagcgtttggacctagtccctcttcctctcgccagtcgtctccaagaaggacggaagatcaagaaggcaaagctcacctcagtgctgcgcagcctcgggcacgaacagccgcctagcgcaccctcatggcgcccggcgcccggcggcgccaccagcccagggtggacatctcccgcgcctcccaaacctctcctcccgcagctgcccagacttctgc

SEQ ID NO: 16586 - RNA, 2064 nt, Homo sapiens
  source 1..2064: mol_type = other RNA
gtgggctgggctgggctgggcctaaaggtttccccgcgctcacgttcacgttcacgttcatgttcacgctcattatctttgtcatccccaaagtggattttctggtgctcaatcagggcagaactatgaaggaaggtttccttacacaccctgcactcgtagaatttgtctttgccatatattttctgaagctcactaaaggtggggctaggcatgaaggcttcctcacattcctgattcttacattccacaagataacctctagcatgaatcttccgatgttcagccaaggcggcactcttattgaaggtctctccacagtccttacattcaaaacgtttccctccaacctgacttttctgaacttcactgacagccacactgtggataaaggactcaccatactcatagaggttctctctagtatgcatgatctggtgctcaacaaattctgagatgacactgaacgacctcccacactcatcacatacatatggcattgccccaaaatcaattggctgtgactcggtaaaggagggggagctgaggctgctcaggctgctcacgctcatggcttttctcatctcactaccacattcaaagggcttcttcctgggacagcctttttgatcgtgaatcgagcccttcccatctgtgtcaaaatgatagcgcctctttctttcaagaactctctttctggaaacaagggttgaattaaacctaaagcctcccctaaatgcattcccttcataaacccgctgctggatcactgactccctcttgttcaatgaaatgtccttccagttatcatctgacattctggggaatctctgtgaccggtcgcttgactcccttgctcttcccgatttggaactgcgtgacacatccttgatgaatttttccattatcactccgtgggaagattcatcttcacaaatcccccgccggtgggttgattttttggcttcaggcatagtttttagacctcgactggtgcttgggtaggcacttctcttggatcttgatgagtggccctgcgtcatgtgggagtggccatcgtcttcagcaagctgcactccgagggagagcagcttcctgtagttttccatgttgtcctggattgtgttgtgaggtttcctgtcctcagcgaggtccaccacattttggtatgattcagcatcctgagatcgggactcataagccctggagtccctgtcgtcctctctgtccatttcaaagcttgttttcgccaccacaggaagggaaagatcccgcggaggcatcctgcttcttgggttcctggtgtgggaccagcggtctcgtggctccatgtctctgcttctgcccctccggtcccagtcccggtcaccactgaaagaatggactgagtgaggtggtgaggactctcttctgttccgggtcatgtcgtcgtcgctggtcacgtcactgttgttgtcgtcttctggttggtacatctccttgtaattctccagcagagtgacgagcttctcacagttctccggcttttttgctcgcacccaaggcttgagcttttcagggatgatggtcaggtactgctcaaggaccaagagctcgatgatctcctccttggtgcgggtctccggctgtctgggaacaggatcctttctggaacttcagaccaagcagctatccacaggaacagagtcaaaacacaggtatctcattaaaagggggctggaattgagaactttaaagtcaggaaccgaggaggttactctcttcgtctcccagggacagcgtggtgtgtggtctcgtctctcttcttgtttgctccattctcctgcctctctctggacccagccacctagcgtttggacctagtccctcttcctctcgccagtcgtctccaagaaggacggaagatcaagaaggcaaagctcacctcagtgctgcgcagcctcgggcacgaacagccgcctagcgcaccctcatggcgcccggcgcccggcggcgccaccagcccagggtggacatctcccgcgcctcccaaacctctcctcccgcagctgcccagacttctgc

SEQ ID NO: 16587 - RNA, 2185 nt, Homo sapiens
  source 1..2185: mol_type = other RNA
gtgggctgggctgggctgggcctaaaggtttccccgcgctcacgttcacgttcacgttcatgttcacgctcattatctttgtcatccccaaagtggattttctggtgctcaatcagggcagaactatgaaggaaggtttccttacacaccctgcactcgtagaatttgtctttgccatatattttctgaagctcactaaaggtggggctaggcatgaaggcttcctcacattcctgattcttacattccacaagataacctctagcatgaatcttccgatgttcagccaaggcggcactcttattgaaggtctctccacagtccttacattcaaaacgtttccctccaacctgacttttctgaacttcactgacagccacactgtggataaaggactcaccatactcatagaggttctctctagtatgcatgatctggtgctcaacaaattctgagatgacactgaacgacctcccacactcatcacatacatatggcattgccccaaaatcaattggctgtgactcggtaaaggagggggagctgaggctgctcaggctgctcacgctcatggcttttctcatctcactaccacattcaaagggcttcttcctgggacagcctttttgatcgtgaatcgagcccttcccatctgtgtcaaaatgatagcgcctctttctttcaagaactctctttctggaaacaagggttgaattaaacctaaagcctcccctaaatgcattcccttcataaacccgctgctggatcactgactccctcttgttcaatgaaatgtccttccagttatcatctgacattctggggaatctctgtgaccggtcgcttgactcccttgctcttcccgatttggaactgcgtgacacatccttgatgaatttttccattatcactccgtgggaagattcatcttcacaaatcccccgccggtgggttgattttttggcttcaggcatagtttttagacctcgactggtgcttgggtaggcacttctcttggatcttgatgagtggccctgcgtcatgtgggagtggccatcgtcttcagcaagctgcactccgagggagagcagcttcctgtagttttccatgttgtcctggattgtgttgtgaggtttcctgtcctcagcgaggtccaccacattttggtatgattcagcatcctgagatcgggactcataagccctggagtccctgtcgtcctctctgtccatttcaaagcttgttttcgccaccacaggaagggaaagatcccgcggaggcatcctgcttcttgggttcctggtgtgggaccagcggtctcgtggctccatgtctctgcttctgcccctccggtcccagtcccggtcaccactgaaagaatggactgagtgaggtggtgaggactctcttctgttccgggtcatgtcgtcgtcgctggtcacgtcactgttgttgtcgtcttctggttggtacatctccttgtaattctccagcagagtgacgagcttctcacagttctccggcttttttgctcgcacccaaggcttgagcttttcagggatgatggtcaggtactgctcaaggaccaagagctcgatgatctcctccttggtgcgggtctccggctgtctgggaacaggatcctttctggaacttcagaccaagcagctatccacaggaacagagtcaaaacacaggtatctcattaaaagggggctggaattgagaactttaaagtcaggaaccgaggaggttactctcttcgtctcccagggacagcgtggtgtgtggtctcgtctctcttcttgtttgctccattctcctgcctctctctttccaggtgggatgactcaggaggtctgtggttccccaggaaagaagcattcctacaatcactccaggagctgttctttgagaaccactgctctaaggtatccagtctggtccaatcacctggacccagccacctagcgtttggacctagtccctcttcctctcgccagtcgtctccaagaaggacggaagatcaagaaggcaaagctcacctcagtgctgcgcagcctcgggcacgaacagccgcctagcgcaccctcatggcgcccggcgcccggcggcgccaccagcccagggtggacatctcccgcgcctcccaaacctctcctcccgcagctgcccagacttctgc

SEQ ID NO: 16588 - RNA, 2180 nt, Homo sapiens
  source 1..2180: mol_type = other RNA
gtgggctgggctgggctgggcctaaaggtttccccgcgctcacgttcacgttcacgttcatgttcacgctcattatctttgtcatccccaaagtggattttctggtgctcaatcagggcagaactatgaaggaaggtttccttacacaccctgcactcgtagaatttgtctttgccatatattttctgaagctcactaaaggtggggctaggcatgaaggcttcctcacattcctgattcttacattccacaagataacctctagcatgaatcttccgatgttcagccaaggcggcactcttattgaaggtctctccacagtccttacattcaaaacgtttccctccaacctgacttttctgaacttcactgacagccacactgtggataaaggactcaccatactcatagaggttctctctagtatgcatgatctggtgctcaacaaattctgagatgacactgaacgacctcccacactcatcacatacatatggcattgccccaaaatcaattggctgtgactcggtaaaggagggggagctgaggctgctcaggctgctcacgctcatggcttttctcatctcactaccacattcaaagggcttcttcctgggacagcctttttgatcgtgaatcgagcccttcccatctgtgtcaaaatgatagcgcctctttctttcaagaactctctttctggaaacaagggttgaattaaacctaaagcctcccctaaatgcattcccttcataaacccgctgctggatcactgactccctcttgttcaatgaaatgtccttccagttatcatctgacattctggggaatctctgtgaccggtcgcttgactcccttgctcttcccgatttggaactgcgtgacacatccttgatgaatttttccattatcactccgtgggaagattcatcttcacaaatcccccgccggtgggttgattttttggcttcaggcatagtttttagacctcgactggtgcttgggtaggcacttctcttggatcttgatgagtggccctgcgtcatgtgggagtggccatcgtcttcagcaagctgcactccgagggagagcagcttcctgtagttttccatgttgtcctggattgtgttgtgaggtttcctgtcctcagcgaggtccaccacattttggtatgattcagcatcctgagatcgggactcataagccctggagtccctgtcgtcctctctgtccatttcaaagcttgttttcgccaccacaggaagggaaagatcccgcggaggcatcctgcttcttgggttcctggtgtgggaccagcggtctcgtggctccatgtctctgcttctgcccctccggtcccagtcccggtcaccactgaaagaatggactgagtgaggtggtgaggactctcttctgttccgggtcatgtcgtcgtcgctggtcacgtcactgttgttgtcgtcttctggttggtacatctccttgtaattctccagcagagtgacgagcttctcacagttctccggcttttttgctcgcacccaaggcttgagcttttcagggatgatggtcaggtactgctcaaggaccaagagctcgatgatctcctccttggtgcgggtctccggctgtctgggaacaggatcctttctggaacttcagaccaagcagctatccacaggaacagagtcaaaacacaggtatctcattaaaagggggctggaattgagaactttaaagtcaggaaccgaggaggttactctcttcgtctcccagggacagcgtggtgtgtggtctcgtctctcttcttgtttgctccattctcctgcctctctctttccaggtgggatgactcaggaggtctgtggttccccaggaaagaagcattcctacaatcactccaggagctgttctttgagaaccactgctctaaggtatccagtctggtccaatcacctggacccagccacctagcgtttggacctagtccctcttcctctcgccagtcgtctccaagaaggacggaagatcaagaaggcaaagctcagtgctgcgcagcctcgggcacgaacagccgcctagcgcaccctcatggcgcccggcgcccggcggcgccaccagcccagggtggacatctcccgcgcctcccaaacctctcctcccgcagctgcccagacttctgc

SEQ ID NO: 16589 - RNA, 1933 nt, Homo sapiens
  source 1..1933: mol_type = other RNA
gtgggctgggctgggctgggcctaaaggtttccccgcgctcacgttcacgttcacgttcatgttcacgctcattatctttgtcatccccaaagtggattttctggtgctcaatcagggcagaactatgaaggaaggtttccttacacaccctgcactcgtagaatttgtctttgccatatattttctgaagctcactaaaggtggggctaggcatgaaggcttcctcacattcctgattcttacattccacaagataacctctagcatgaatcttccgatgttcagccaaggcggcactcttattgaaggtctctccacagtccttacattcaaaacgtttccctccaacctgacttttctgaacttcactgacagccacactgtggataaaggactcaccatactcatagaggttctctctagtatgcatgatctggtgctcaacaaattctgagatgacactgaacgacctcccacactcatcacatacatatggcattgccccaaaatcaattggctgtgactcggtaaaggagggggagctgaggctgctcaggctgctcacgctcatggcttttctcatctcactaccacattcaaagggcttcttcctgggacagcctttttgatcgtgaatcgagcccttcccatctgtgtcaaaatgatagcgcctctttctttcaagaactctctttctggaaacaagggttgaattaaacctaaagcctcccctaaatgcattcccttcataaacccgctgctggatcactgactccctcttgttcaatgaaatgtccttccagttatcatctgacattctggggaatctctgtgaccggtcgcttgactcccttgctcttcccgatttggaactgcgtgacacatccttgatgaatttttccattatcactccgtgggaagattcatcttcacaaatcccccgccggtgggttgattttttggcttcaggcatagtttttagacctcgactggtgcttgggtaggcacttctcttggatcttgatgagtggccctgcgtcatgtgggagtggccatcgtcttcagcaagctgcactccgagggagagcagcttcctgtagttttccatgttgtcctggattgtgttgtgaggtttcctgtcctcagcgaggtccaccacattttggtatgattcagcatcctgagatcgggactcataagccctggagtccctgtcgtcctctctgtccatttcaaagcttgttttcgccaccacaggaagggaaagatcccgcggaggcatcctgcttcttgggttcctggtgtgggaccagcggtctcgtggctccatgtctctgcttctgcccctccggtcccagtcccggtcaccactgaaagaatggactgagtgaggtggtgaggactctcttctgttccgggtcatgtcgtcgtcgctggtcacgtcactgttgttgtcgtcttctggttggtacatctccttgtaattctccagcagagtgacgagcttctcacagttctccggcttttttgctcgcacccaaggcttgagcttttcagggatgatggtcaggtactgctcaaggaccaagagctcgatgatctcctccttggtgcgggtctccggctgtctgggaacaggatcctttctggaacttcagaccaagcagctatccacaggaacagagtcaaaacacaggtatctggacccagccacctagcgtttggacctagtccctcttcctctcgccagtcgtctccaagaaggacggaagatcaagaaggcaaagctcacctcagtgctgcgcagcctcgggcacgaacagccgcctagcgcaccctcatggcgcccggcgcccggcggcgccaccagcccagggtggacatctcccgcgcctcccaaacctctcctcccgcagctgcccagacttctgc

SEQ ID NO: 16590 - RNA, 1928 nt, Homo sapiens
  source 1..1928: mol_type = other RNA
gtgggctgggctgggctgggcctaaaggtttccccgcgctcacgttcacgttcacgttcatgttcacgctcattatctttgtcatccccaaagtggattttctggtgctcaatcagggcagaactatgaaggaaggtttccttacacaccctgcactcgtagaatttgtctttgccatatattttctgaagctcactaaaggtggggctaggcatgaaggcttcctcacattcctgattcttacattccacaagataacctctagcatgaatcttccgatgttcagccaaggcggcactcttattgaaggtctctccacagtccttacattcaaaacgtttccctccaacctgacttttctgaacttcactgacagccacactgtggataaaggactcaccatactcatagaggttctctctagtatgcatgatctggtgctcaacaaattctgagatgacactgaacgacctcccacactcatcacatacatatggcattgccccaaaatcaattggctgtgactcggtaaaggagggggagctgaggctgctcaggctgctcacgctcatggcttttctcatctcactaccacattcaaagggcttcttcctgggacagcctttttgatcgtgaatcgagcccttcccatctgtgtcaaaatgatagcgcctctttctttcaagaactctctttctggaaacaagggttgaattaaacctaaagcctcccctaaatgcattcccttcataaacccgctgctggatcactgactccctcttgttcaatgaaatgtccttccagttatcatctgacattctggggaatctctgtgaccggtcgcttgactcccttgctcttcccgatttggaactgcgtgacacatccttgatgaatttttccattatcactccgtgggaagattcatcttcacaaatcccccgccggtgggttgattttttggcttcaggcatagtttttagacctcgactggtgcttgggtaggcacttctcttggatcttgatgagtggccctgcgtcatgtgggagtggccatcgtcttcagcaagctgcactccgagggagagcagcttcctgtagttttccatgttgtcctggattgtgttgtgaggtttcctgtcctcagcgaggtccaccacattttggtatgattcagcatcctgagatcgggactcataagccctggagtccctgtcgtcctctctgtccatttcaaagcttgttttcgccaccacaggaagggaaagatcccgcggaggcatcctgcttcttgggttcctggtgtgggaccagcggtctcgtggctccatgtctctgcttctgcccctccggtcccagtcccggtcaccactgaaagaatggactgagtgaggtggtgaggactctcttctgttccgggtcatgtcgtcgtcgctggtcacgtcactgttgttgtcgtcttctggttggtacatctccttgtaattctccagcagagtgacgagcttctcacagttctccggcttttttgctcgcacccaaggcttgagcttttcagggatgatggtcaggtactgctcaaggaccaagagctcgatgatctcctccttggtgcgggtctccggctgtctgggaacaggatcctttctggaacttcagaccaagcagctatccacaggaacagagtcaaaacacaggtatctggacccagccacctagcgtttggacctagtccctcttcctctcgccagtcgtctccaagaaggacggaagatcaagaaggcaaagctcagtgctgcgcagcctcgggcacgaacagccgcctagcgcaccctcatggcgcccggcgcccggcggcgccaccagcccagggtggacatctcccgcgcctcccaaacctctcctcccgcagctgcccagacttctgc

SEQ ID NO: 16591 - RNA, 1140 nt, Homo sapiens
  source 1..1140: mol_type = other RNA
gtgggctgggctgggctgggcctaggtgtgcgtgggggcggtgctggtctgctttgctgggagccatggacaccggaggaacagggccccatcagtgcggtcagagtgcaaactcggagcgtccttctctggaaaacgaatcgcagtggccccgatctttggggctttctgtgtcccctgtatccctttactccgcgtacacaggtgcctttgtcacttctcctttgacctggctggcacatcttaccggtttctgcgctaacaatgagttgaaggaaatcttgaacgcgcgttcattttatatcggtatcagagtctgtttatttcttgttgacactaatctttgagcatgagtagtttagtgattgtgaaacagaaacttctggatacaaaatcagtctcctggctgtgacccaatcatcttcgcagttctgattacctgcaggctcccagcccaggctactgacatcaatcatggcaatcgctattccagaggtatacgcggtgggtggggtccggtatcgcctgccatgcctcactcaccgggcacccagataacctgaggccagggagcagccactcgccctgacccatgctccccgggcccctgaggcacccaggaggaccacccggccgcttctgctcagagcccagcacccccgagtctgtgaagaggtcacatctgaccacgtttccaggtggctgcccaggcgtgggttcatggccgcttccggtttcctcctcgagctgaaccacacacctgctctgtcccgggctttctggaggggttttccgaagtgagactgtgggctccctccagggctgggggcaggaggacacacggggaaggtgggcaagcagccccaggctgagggaggcctcccctctgcagcgtttgttcattcatttgttcatcgctaacactgtcttgggcatcagggaaaacaggtgtctctggtccacatgcagaagagccaccaccgtggcacgactggatgactcagaccccgggcggggggtatgatttggacacagtcattgtccagggacacaactttgcctggaccagagcttctcacccccaggccatttgaaaccccaggggatactcgacaaagtccagagacattttgggttgtt

SEQ ID NO: 16592 - RNA, 1141 nt, Homo sapiens
  source 1..1141: mol_type = other RNA
gtgggctgggctgggctgggcctaggtgtgcgtgggggcggtgctggtctgctttgctgggagccatggacaccggaggaacagggccccatcagtgcggtcagagtgcaaactcggagcgtccttctctggaaaacgaatcgcagtggccccgatctttggggctttctgtgtcccctgtatccctttactccgcgtacacaggtgcctttgtcacttctcctttgacctggctggcacatcttaccggtttctgcgctaacaatgagttgaaggaaatcttgaacgcgcgttcattttatatcggtatcagagtctgtttatttcttgttgacactaatctttgagcatgagtagtttagtgattgtgaaacagaaacttctggatacaaaatcagtctcctggctgtgacccaatcatcttcgcagttctgattacctgcaggctcccagcccaggctactgacatcaatcatggcaatcgctattccagaggtatacgcggtgggtggggtccggtatcgcctgccatgcctcactcaccgggcacccagataacctgaggccagggagcagccactcgccctgacccatgctccccgggcccctgaggcacccaggaggaccacccggccgcttctgctcagagcccagcacccccgagtctgtgaagaggtcacatctgaccacgtttccaggtggctgcccaggcgtgggttcatggccgcttccggtttcctcctcgagctgaaccacacacctgctctgtcccgggctttctggaggggttttccgaagtgagactgtgggctccctccagggctgggggcaggaggacacacggggaaggtgggcaagcagccccaggctgagggaggcctcccctctgcagcgtttgttcattcatttgttcatcgctaacactgtcttgggcatcagggaaaacaggtgtctctggtccacatgcagaagagccaccaccgtggcacgactggatgactcagaccccgggcggggggtatgatttggacacagtcattgtccagggacacaactttgcctggaccagagcttctcacccccaggccatttgaaaccccaggggatactcgacaaagtccagagacattttgggttgttc

SEQ ID NO: 16593 - RNA, 1440 nt, Homo sapiens
  source 1..1440: mol_type = other RNA
gtgggctgggctgggctgggcctaggtgtgcgtgggggcggtgctggtctgctttgctgggagccatggacaccggaggaacagggccccatcagtgcggtcagagtgcaaactcggagcgtccttctctggaaaacgaatcgcagtggccccgatctttggggctttctgtgtcccctgtatccctttactccgcgtacacaggtgcctttgtcacttctcctttgacctggctggcacatcttaccggtttctgcgctaacaatgagttgaaggaaatcttgaacgcgcgttcattttatatcggtatcagagtctgtttatttcttgttgacactaatctttgagcatgagtagtttagtgattgtgaaacagaaacttctggatacaaaatcagtctcctggctgtgacccaatcatcttcgcagttctgattacctgcaggctcccagcccaggctactgacatcaatcatggcaatcgctattccagaggtatacgcggtgggtggggtccggtatcgcctgccatgcctcactcaccgggcacccagataacctgaggccagggagcagccactcgccctgacccatgctccccgggcccctgaggcacccaggaggaccacccggccgcttctgctcagagcccagcacccccgagtctgtgaagaggtcacatctgaccacgtttccaggtggctgcccaggcgtgggttcatggccgcttccggtttcctcctcgagctgaaccacacacctgctctgtcccgggctttctggaggggttttccgaagtgagactgtgggctccctccagggctgggggcaggaggacacacggggaaggtgggcaagcagccccaggctgagggaggcctcccctctgcagcgtttgttcattcatttgttcatcgctaacactgtcttgggcatcagggaaaacaggtgtctctggtccacatgcagaagagccaccaccgtggcacgactggatgactcagaccccgggcggggggtatgatttggacacagtcattgtccagggacacaactttgcctggaccagagcttctcacccccaggccatttgaaaccccaggggatactcgacaaagtccagagacattttgggttgttcctttccagccccggcgatggtggggacgtgtccatgtctgtgtccctccggtcactctctctggccctctccctccctgggggcagctgctctcagccctccctgcccccacatcgccatcctgcctgtccttctgggcctgcacgtttgttgtgtttggaaggagccaccaaggaggaggatgtcaatgtgcaagttctcagggaagcaggccccgcagcctccgtcagtgtcttccgtccgcaggaagaacccaggcctgggtgattcatcggggcctcagggccgggaggcactaa

SEQ ID NO: 16594 - RNA, 1648 nt, Homo sapiens
  source 1..1648: mol_type = other RNA
gtgggctgggctgggctgggcctcagcaaggtgacatttcatgtctagaaatagcagcaagtgctcagttaattggtcaataaaggggagaaatttgcttacaaaaaaggctggcttgctgggaggccacctggcgggccagccctgtgtcagaggaggggccaggtgggtccctcagcccccagagagggagctgtgcggtcggcagtgggaggctccgaaggcaccagccctcccttgacgccctggccccacttcctcggaaaccccagcagccccgagccgcccacccaggggcagctccctcgtgtgaggtgcagggtggagccgggcctgggtcagaactgagcgtggtctacctcatccagccaggaggcggggctggcagggaagtcggggtaacccccgctgctccccgtggataggtcagaactgggtccgttccctgccagcaccctcatgggtgggggcccgccgggggctcccgagggcacaaggcccaagctggtgtctgggtacaccaggctggagaggaggggctgggggccagggaggctctgcggggcggcgggggatggggggacaccgtaggggctgccgggacgcagctctcggtactgctctgggcctgccaggcctccatgctccagggagaagttgcccagggctcccgagggccggcccaaggcctgggtgggttcccccaagctcccgtagaggccattggccgggcccatttccgccaaggaaggctcatcggggaaggagacctcagcgtcgctgtcctgcccctcctgaacgctgtccttgtccgacttggagccgccgcgggagcgcttcatgttgcggaaatactgcccccagcgctgccggccggcgtccttcttcagcctcttctccttggcccggcggttctggaaccaaacctgcaccacgcgcatgtccaggcccgtctcggacgagagctgctcgcgcacgtggcgcgccggcttgggcgaggtgttgtaagcgctcttcagcgtctccagctgcttggcggtgatggtcgtgcgcggccgcttggccgtggcctcggcctctcgctgcttggcggtttcgtagtccgccttgcacacgagccggctgtcctccatgaggtagaactcgtcgcccgtggccagctgccgcttgcacacgacgcaggcaaagcagtgcaggtggtacacgaagtcctgggcgcggcgcaccacctgcgtgggcgggatgcccagctggcacgcggcgcacttggtcccgaagcgcttgaaaaagtcgtccttgcagtaaacgctctcccctcggctgaagcagcgctcggccagtggcgtgtggcagtcgctgcacttgagacacttgctgtgccagtggcggtccagagccttgaggatgaagcggtccaggatgtgctggtcacagccagcgcacagcgggatctcccgagtcccgcccaaggtgcagacggcggcggccccgggcctcgctcggtcgcgctcgagccccgtttccagcagcatcgcggccaccaggccgagtggcgcgagacgcgctcctcctaggtcagcgtcccctggagggttcggggctcccaagtcccgccgcgtcgtgcggggcagggagcccgggagccact

SEQ ID NO: 16595 - RNA, 1697 nt, Homo sapiens
  source 1..1697: mol_type = other RNA
gtgggctgggctgggctgggcctcagcaaggtgacatttcatgtctagaaatagcagcaagtgctcagttaattggtcaataaaggggagaaatttgcttacaaaaaaggctggcttgctgggaggccacctggcgggccagccctgtgtcagaggaggggccaggtgggtccctcagcccccagagagggagctgtgcggtcggcagtgggaggctccgaaggcaccagccctcccttgacgccctggccccacttcctcggaaaccccagcagccccgagccgcccacccaggggcagctccctcgtgtgaggtgcagggtggagccgggcctgggtcagaactgagcgtggtctacctcatccagccaggaggcggggctggcagggaagtcggggtaacccccgctgctccccgtggataggtcagaactgggtccgttccctgccagcaccctcatgggtgggggcccgccgggggctcccgagggcacaaggcccaagctggtgtctgggtacaccaggctggagaggaggggctgggggccagggaggctctgcggggcggcgggggatggggggacaccgtaggggctgccgggacgcagctctcggtactgctctgggcctgccaggcctccatgctccagggagaagttgcccagggctcccgagggccggcccaaggcctgggtgggttcccccaagctcccgtagaggccattggccgggcccatttccgccaaggaaggctcatcggggaaggagacctcagcgtcgctgtcctgcccctcctgaacgctgtccttgtccgacttggagccgccgcgggagcgcttcatgttgcggaaatactgcccccagcgctgccggccggcgtccttcttcagcctcttctccttggcccggcggttctggaaccaaacctgcaccacgcgcatgtccaggcccgtctcggacgagagctgctcgcgcacgtggcgcgccggcttgggcgaggtgttgtaagcgctcttcagcgtctccagctgcttggcggtgatggtcgtgcgcggccgcttggccgtggcctcggcctctcgctgcttggcggtttcgtagtccgccttgcacacgagccggctgtcctccatgaggtagaactcgtcgcccgtggccagctgccgcttgcacacgacgcaggcaaagcagtgcaggtggtacacgaagtcctgggcgcggcgcaccacctgcgtgggcgggatgcccagctggcacgcggcgcacttggtcccgaagcgcttgaaaaagtcgtccttgcagtaaacgctctcccctcggctgaagcagcgctcggccagtggcgtgtggcagtcgctgcacttgagacacttgctgtgccagtggcggtccagagccttgaggatgaagcggtccaggatgtgctggtcacagccagcgcacagcgggatctctcggcgcaggtccgccctccgcgccagcagtgctagcagcaggtcgcctcccgccgactcccgggccgggcccagctccccgcgcgcctccatgggtcccgccgcccggcgtcgccactctccagtcccgaactttcccgggcccagcgacgccaccccgcaatagccccgaaccggcgtccaagcgactccgggtgctgctgggcgctgcgcccgcgggccgccctggggcccggagcctct

SEQ ID NO: 16596 - RNA, 1963 nt, Homo sapiens
  source 1..1963: mol_type = other RNA
gtgggctgggctgggctgggcctcagcaaggtgacatttcatgtctagaaatagcagcaagtgctcagttaattggtcaataaaggggagaaatttgcttacaaaaaaggctggcttgctgggaggccacctggcgggccagccctgtgtcagaggaggggccaggtgggtccctcagcccccagagagggagctgtgcggtcggcagtgggaggctccgaaggcaccagccctcccttgacgccctggccccacttcctcggaaaccccagcagccccgagccgcccacccaggggcagctccctcgtgtgaggtgcagggtggagccgggcctgggtcagaactgagcgtggtctacctcatccagccaggaggcggggctggcagggaagtcggggtaacccccgctgctccccgtggataggtcagaactgggtccgttccctgccagcaccctcatgggtgggggcccgccgggggctcccgagggcacaaggcccaagctggtgtctgggtacaccaggctggagaggaggggctgggggccagggaggctctgcggggcggcgggggatggggggacaccgtaggggctgccgggacgcagctctcggtactgctctgggcctgccaggcctccatgctccagggagaagttgcccagggctcccgagggccggcccaaggcctgggtgggttcccccaagctcccgtagaggccattggccgggcccatttccgccaaggaaggctcatcggggaaggagacctcagcgtcgctgtcctgcccctcctgaacgctgtccttgtccgacttggagccgccgcgggagcgcttcatgttgcggaaatactgcccccagcgctgccggccggcgtccttcttcagcctcttctccttggcccggcggttctggaaccaaacctgcaccacgcgcatgtccaggcccgtctcggacgagagctgctcgcgcacgtggcgcgccggcttgggcgaggtgttgtaagcgctcttcagcgtctccagctgcttggcggtgatggtcgtgcgcggccgcttggccgtggcctcggcctctcgctgcttggcggtttcgtagtccgccttgcacacgagccggctgtcctccatgaggtagaactcgtcgcccgtggccagctgccgcttgcacacgacgcaggcaaagcagtgcaggtggtacacgaagtcctgggcgcggcgcaccacctgcgtgggcgggatgcccagctggcacgcggcgcacttggtcccgaagcgcttgaaaaagtcgtccttgcagtaaacgctctcccctcggctgaagcagcgctcggccagtggcgtgtggcagtcgctgcacttgagacacttgctgtgccagtggcggtccagagccttgaggatgaagcggtccaggatgtgctggtcacagccagcgcacagcgggatctctggagctggggcaccccatcgggtctccttcatgttaagcgtcatggccactctttctagggactcctcgcaaatgtggctgccctgcctggtggccctgtctgcaggcctccggggtaaatatcaatgccttccccatcattgggcagccgcaaaattacttatgagtggactggacaagccgatccactgcctttgtgtcaggcgtgggtgcccccaacaccgtcagagttactcaaacgtctggcttcccgctgcttctgccccccacaccccacttcggtactgcaggccccctggaggaaccacactggggaggtccaagggtgccctgtgggagcctcgagtctgtgagcgggttttccaggtgtcaagggctgaggactccctcttcacttagaaaaagtctctggaagagaggagtgcccgctgaagggaccgggatttactgacatattgcacccgcctccctggctgtggaccccgccggctccagcccatctcccagt

SEQ ID NO: 16597 - RNA, 1460 nt, Homo sapiens
  source 1..1460: mol_type = other RNA
gtgggctgggctgggctgggcctcagcaaggtgacatttcatgtctagaaatagcagcaagtgctcagttaattggtcaataaaggggagaaatttgcttacaaaaaaggctggcttgctgggaggccacctggcgggccagccctgtgtcagaggaggggccaggtgggtccctcagcccccagagagggagctgtgcggtcggcagtgggaggctccgaaggcaccagccctcccttgacgccctggccccacttcctcggaaaccccagcagccccgagccgcccacccaggggcagctccctcgtgtgaggtgcagggtggagccgggcctgggtcagaactgagcgtggtctacctcatccagccaggaggcggggctggcagggaagtcggggtaacccccgctgctccccgtggataggtcagaactgggtccgttccctgccagcaccctcatgggtgggggcccgccgggggctcccgagggcacaaggcccaagctggtgtctgggtacaccaggctggagaggaggggctgggggccagggaggctctgcggggcggcgggggatggggggacaccgtaggggctgccgggacgcagctctcggtactgctctgggcctgccaggcctccatgctccagggagaagttgcccagggctcccgagggccggcccaaggcctgggtgggttcccccaagctcccgtagaggccattggccgggcccatttccgccaaggaaggctcatcggggaaggagacctcagcgtcgctgtcctgcccctcctgaacgctgtccttgtccgacttggagccgccgcgggagcgcttcatgttgcggaaatactgcccccagcgctgccggccggcgtccttcttcagcctcttctccttggcccggcggttctggaaccaaacctgcaccacgcgcatgtccaggcccgtctcggacgagagctgctcgcgcacgtggcgcgccggcttgggcgaggtgttgtaagcgctcttcagcgtctccagctgcttggcggtgatggtcgtgcgcggccgcttggccgtggcctcggcctctcgctgcttggcggtttcgtagtccgccttgcacacgagccggctgtcctccatgaggtagaactcgtcgcccgtggccagctgccgcttgcacacgacgcaggcaaagcagtgcaggtggtacacgaagtcctgggcgcggcgcaccacctgcgtgggcgggatgcccagctggcacgcggcgcacttggtcccgaagcgcttgaaaaagtcgtccttgcagtaaacgctctcccctcggctgaagcagcgctcggccagtggcgtgtggcagtcgctgcacttgagacacttgctgtgccagtggcggtccagagccttgaggatgaagcggtccaggatgtgctggtcacagccagcgcacagcgggatctgctgcat

SEQ ID NO: 16598 - RNA, 2839 nt, Homo sapiens
  source 1..2839: mol_type = other RNA
gtgggctgggctgggctgggcctccggacaggggcatgagctgggccactggctgaccaggggtgtccgtcatccaggggtgtccgtcatccaggggtgtccatccatccccagtgggcacagctccaacccctccagggcagcctcagctcccattcccatccagtctgcccctgcccagcctgcccagctgggtgcaggccatgccctcaggcccaagtgggcctagcctcattctctgtgggtggctcacccctcttcccagggtgggctgccccccgtcctccccacaggggaagatcctatgtctgggcccaccgtggacagccggaggagacctcacaccctctcctggaggccacgctggtgcgtgtggccaggtgtgggatctgggcctcgctggctaccaggacatactgtcatccttgtgtgctgggggacggggctgtccctgacatgaggaaagaggcaggcaacttcagtacacggtgctggatgggaggagatgagaggagaaccctggcactcgagacctccctccaagacgcccttgccgccgagtccgtcctgaacctcggcgagtgagtcactttcccactcagaggtcagtttctccgaagtgacttcccagagccgtgaagacagcaagccagcctctggcaagcgatggcttgggggcagcggtgagggaggggctgtgctgagcaacctcaggactggtcgccagtgcctgagtcagggcacctggatggggtcacaggcagggaggtgggcacgtctccagctgcgcagccccgtctacccagcccagccccagagaccctaccagcctggcaggagggcagtgtggcttagagcaggtaggagatggatctgatggcgagtgccgggctctttgtgcataaaacgggccccagatactcacagtgggccctcgtgtgctgtctcagtcgtggtcccgtgggaggaacgtgagtgtcgggaaccagtagcaagagggagggccagggagcagggcctgggctggggaagaacctgaaaggggtgctggagtggctgccctgtgggaggcggagggaggggcctctaaagaagcacggccgattgctgcgactctgggcctcctggtttttaagaccacagcagacaattaaactgcccctcactcgtgtttggcggtctctggccgcacggaagccaggggtcagagccctaccagcccaggcagagtcagttccttgaggtcaggccctccaggacctgggggatccagggaccaagtgggtggacagctctgctcctggggtgatcttccccctcccctgagtcctgacccaaataaacagctggtgccctgtccttgcagcctatgctcctggggagccggcctgggatttggatttgtactcatgaaggacagcgctccctgactcccagctccccctccctgggctgctccccttggcagatcaccaggggagggggacaggatgcgggaaccagcgccctccctctcctgaggctcagcagagccctgcccggtcccgcagtgctcccaggaccctgtaccagcccatctgtgcactgtgcctcgggcactcctggtaacgatgcctcttcctccaggacgtgcgcccaggcctccgctcagcgccgtccgggtttcctgctgcctcctcttgctcctttcggggacacaagacacccgggtcttgctcctgccataccctgctctgaacctccccccaggaaccccgaccagaccgccaggcagtgcctggactcgctgtccagagtggggaattcgaccagactcattcatgtctaaaccctctgagtgtttccaaatcaccccactcccagccccaccgagaggaaggtggggaaagaaaccaagcacggtggagggtccctgctccttccccacaagaggccgcgcctgtggtgccgagtcagcactgctgctggtgtggctgtaaatagtcctgagattggagagctcagctttgaggaggctggaaggtaacaacacctgacaagttttatttttaaatgtatctgcccaggctgcaagaggggcttacataattcaggccagtgtgtttacttagtctaaggtgaaacccaaaaaaagaaaaggagggagggaggaggaagggtgggaaggaagaacagaacagggaagggggagaggaagggtccccagcagcctcggctggcacagacttggctggggctgccctcagccaccgcctggagggagtcaatgtccaccacaggtgtgggggcacctggttggcctcccagcaggctgtttcctggctagggcccttgagcagagccctcaggccacacgtgattcgctgaagtgggcatatcaaggagggggcacgtcctacctggggtgagggccgaacctgctgctcccaggtcagcacagctagtggggaggaggcgtcctgacccctccgtcgattcagggaaatgcgcatatgcagacacaggcacatgcaaacacatgtaaacacatgcaaacacatataaacacgcgtgaacggcagaacagcaggaaggtaacgccagagagaattgggaacagcaggaaggtaatgcgtgaggagaagtgggaatggcaggaaggtaatggcatgaggagaagtaggaacagcatgaaggtaacgccagtgagaagtgggaacagagggaaggtaacgtcgttgaggagaagtaggaatggcgggaaggtaacgctggtgagaagtgggaaaggcgggaaggaaacaccattgaggagaagtgggaacggcaggaaggtaacgccgtgaggagaagtgggaat

SEQ ID NO: 16599 - RNA, 367 nt, Homo sapiens
  source 1..367: mol_type = other RNA
gtgggctgggctgggctgggcctgctggaaggaggcctggcagatgaagatgggcttcccatgttgcacggccttcacagagcgcaccgagaagctcgaccctgttcgtgtccgctccacttggtacagtactggcagcttcgggtcccctgaagagatcctcgtccagcggctcgaggttgagcacggtcgtgaccaagacgctacggaggtccccagggggatcgccgcggtcgccacagccctgcccatcttctggggcctgcggggacgacatctagttcaatgctgcaggccctgcacacccgctccgcggaagacgcggagacatacacagaacctgactcttccggcagattgccctagt

SEQ ID NO: 16600 - RNA, 488 nt, Homo sapiens
  source 1..488: mol_type = other RNA
gtgggctgggctgggctgggcctgctggaaggaggcctggcagatgaagatgggcttcccatgttgcacggccttcacagagcgcaccgagaagctcgaccctgttcgtgtccgctccacttggtacagtactggcagcttcgggtcccctgcccgaacaaagtagcagtgcagggagtgcacgtggacgtcttcactcacagacttggctgcagccaccagggcctggcccacgatctgaccaccaaacagcctcttggccggtacccagtaatgccttcctctgaagagatcctcgtccagcggctcgaggttgagcacggtcgtgaccaagacgctacggaggtccccagggggatcgccgcggtcgccacagccctgcccatcttctggggcctgcggggacgacatctagttcaatgctgcaggccctgcacacccgctccgcggaagacgcggagacatacacagaacctgactcttccggc

SEQ ID NO: 16601 - RNA, 501 nt, Homo sapiens
  source 1..501: mol_type = other RNA
gtgggctgggctgggctgggcctgctggaaggaggcctggcagatgaagatgggcttcccatgttgcacggccttcacagagcgcaccgagaagctcgaccctgttcgtgtccgctccacttggtacagtactggcagcttcgggtcccctgcccgaacaaagtagcagtgcagggagtgcacgtggacgtcttcactcacagacttggctgcagccaccagggcctggcccacgatctgaccaccaaacagcctcttggccggtacccagtaatgccttcctctgaagagatcctcgtccagcggctcgaggttgagcacggtcgtgaccaagacgctacggaggtccccagggggatcgccgcggtcgccacagccctgcccatcttctggggcctgcggggacgacatctagttcaatgctgcaggccctgcacacccgctccgcggaagacgcggagacatacacagaacctgactcttccggcagattgccctagt

SEQ ID NO: 16602 - RNA, 529 nt, Homo sapiens
  source 1..529: mol_type = other RNA
gtgggctgggctgggctgggcctgctggaaggaggcctggcagatgaagatgggcttcccatgttgcacggccttcacagagcgcaccgagaagctcgaccctgttcgtgtccgctccacttggtacagtactggcagcttcgggtccctgtaaaggtccacaaactcttctcagctggggatctacgcagaacacatgagggcatctgctctgcccgaacaaagtagcagtgcagggagtgcacgtggacgtcttcactcacagacttggctgcagccaccagggcctggcccacgatctgaccaccaaacagcctcttggccggtacccagtaatgccttcctctgaagagatcctcgtccagcggctcgaggttgagcacggtcgtgaccaagacgctacggaggtccccagggggatcgccgcggtcgccacagccctgcccatcttctggggcctgcggggacgacatctagttcaatgctgcaggccctgcacacccgctccgcggaagacgcggagacatac

SEQ ID NO: 16603 - RNA, 2200 nt, Homo sapiens
  source 1..2200: mol_type = other RNA
gtgggctgggctgggctgggcctggggccagacctcaatgactgtttccttcccgtcagcgagcggagaagcagtgacagagtgtaccaggaggggaagctgacggtggccccaactcctctcttgaatgggatatgaccaccccacctgcccctcagtgtttgcaggacactctggcacactcatgccttcctttcctggtgaacctgtatcccactacaaagaggaacagaactccccacccagccccacccttgcttccaggggctttgagacactcaggagaaggagcttcaaatattgtgagggtctgtctgtgtcagccaccaggatgtcaatccctgcctgggctggcagcatggaccttgtggaccctcctagcccaccccatgcccccaggagccccgcttggcttcttctcttttatacattgtaaacaccacatttatttgtctgaggcttgcaaacctctggtaagaagcacagaacgcagggctctccttcatgctgccctgggccccagctcgccaggcatgcaggacagagctggcagatgagtcagaaatctttgggagcagcgccagggaagcagcaggccctgctccttcccatgcccaatcccgccagcacgggcctggactgcagccaggaaggtgggccagccaggatccccaggtaacttcgccacagggacctcttcttggagctgccttcccttccctccccatccctctccaatccccgcagagcttagagcctgggccacatgcttggtccctcacacaaggaccaaaccagctgctgtcaggctgtttctgtgggtcctgtctctccagtcaggaagccagcagggcagggcaggcctggctctcctcctggaatcacaccgtgcacccagctcagcgctgggcactcagctggggaccgggatggacaaagccttgtccagagaaccactgtaggggagacgtgcatggcagccggactcagcctcctgcagcctccattcatgggctcttggctgggcctgaaatttgttagggcctcaactctctgtggtgcagatgaacacctcctcctccaagaggcccctcaggcttggtgccaggcttgggactgggctctggaaagtcagccaaggctgctacttcaaggccctgaggacagcctccagcttcatggccatagccaggtcgcccttcaccttcagccgtccactcatgtaggcccccaggggccgcagctctctgcatagcagggcccgcaggtctgcctcggccatctccaccaccacatcagggatgccatcaggcaccccgtgtcccactcttcctcgtcctggccccggggacggggcacctcctgccattgagttcatgcttcctcccaggaagtgcagggccagctgctggagggtgctgtccaggttgggcccagctgggctgtcctggggcggctggagcacggcctccactgccagctccacgcggtctacctccagcccccaggccctggtcacatcgttgatctccagcagaagctggtcgctgatcttgagcttctccatctggatctcccgcagcggcctcttgagcagggccttggtcatggcgttctgggctgtcatgcgtgtggctgtgttcaggtctttcacagtcatcaccgacagcaccgggtcccagatgcgaaactggacatcggctcccacggacagcacagccccgtccttagaggccagcttgcagggagggacgttgaaggctcgtgtcctcagatccaccctctgaaaggagtcaatgaagggcaagagcagaaccatgccaggtccctggggggtgcggatccggcccaggcggaacacaatcatccgctcgtaggtgggcacaatcttcagggcaaaccagccagaaatggggaaggtgaccaacagcagcaagaaccccaggaaactgatgaggccatgacagaggcaggagggccagctctggggtacatcggcccctgtccccacgccgccccgctccggggacaagcagcccttctgcgagcccagaaagccgaagctcgactgctggaagcggtcaaaatcacccaggggcagcgcccggtacccagacctgccgagcatggcttttgacaggagacacgccccgcgcctccgcgcggcgccctccctggccagtgggccctacgcggcccc

SEQ ID NO: 16604 - RNA, 2718 nt, Homo sapiens
  source 1..2718: mol_type = other RNA
gtgggctgggctgggctgggcctggggccagacctcaatgactgtttccttcccgtcagcgagcggagaagcagtgacagagtgtaccaggaggggaagctgacggtggccccaactcctctcttgaatgggatatgaccaccccacctgcccctcagtgtttgcaggacactctggcacactcatgccttcctttcctggtgaacctgtatcccactacaaagaggaacagaactccccacccagccccacccttgcttccaggggctttgagacactcaggagaaggagcttcaaatattgtgagggtctgtctgtgtcagccaccaggatgtcaatccctgcctgggctggcagcatggaccttgtggaccctcctagcccaccccatgcccccaggagccccgcttggcttcttctcttttatacattgtaaacaccacatttatttgtctgaggcttgcaaacctctggtaagaagcacagaacgcagggctctccttcatgctgccctgggccccagctcgccaggcatgcaggacagagctggcagatgagtcagaaatctttgggagcagcgccagggaagcagcaggccctgctccttcccatgcccaatcccgccagcacgggcctggactgcagccaggaaggtgggccagccaggatccccaggtaacttcgccacagggacctcttcttggagctgccttcccttccctccccatccctctccaatccccgcagagcttagagcctgggccacatgcttggtccctcacacaaggaccaaaccagctgctgtcaggctgtttctgtgggtcctgtctctccagtcaggaagccagcagggcagggcaggcctggctctcctcctggaatcacaccgtgcacccagctcagcgctgggcactcagctggggaccgggatggacaaagccttgtccagagaaccactgtaggggagacgtgcatggcagccggactcagcctcctgcagcctccattcatgggctcttggctgggcctgaaatttgttagggcctcaactctctgtggtgcagatgaacacctcctcctccaagaggcccctcaggcttggtgccaggcttgggactgggctctggaaagtcagccaaggctgctacttcaaggccctgaggacagcctccagcttcatggccatagccaggtcgcccttcaccttcagccgtccactcatgtaggcccccaggggccgcagctctctgcatagcagggcccgcaggtctgcctcggccatctccaccaccacatcagggatgccatcaggcaccccgtgtcccactcttcctcgtcctgtagtgaggtccaggaagtaggcgctttgggtgccgctgggcaggacgacattgaactggtagcaggccccgacttggctgaccagggcctcagacaggaagggctgtagagcagtcagtagcccctccgccagaggctgcttcggactggacctggcaccaacttgaggggcaggtggctcaacttcactcaccatctccacggtgtctgctggccccggggacggggcacctcctgccattgagttcatgcttcctcccaggaagtgcagggccagctgctggagggtgctgtccaggttgggcccagctgggctgtcctggggcggctggagcacggcctccactgccagctccacgcggtctacctccagcccccaggccctggtcacatcgttgatctccagcagaagctggtcgctgatcttgagcttctccatctggatctcccgcagcggcctcttgagcagggccttggtcatggcgttctgggctgtcatgcgtgtggctgtgttcaggtctttcacagtcatcaccgacagcaccgggtcccagatgcgaaactggacatcggctcccacggacagcacagccccgtccttagaggccagctgttgggggaggccatgagagagagacactcaaggggctgggggtgcagggaggtcaggcccactggggccacccagcttgaaccacctgcttggcagctagctcctcaagggcaaatggtgtcaccaagtatgtagggttaggtgtatgaagcaaggatgtcctcctagcttccatcaattttctggtctcttcttcccccttcccccctcagatggtgactcacaggctgaggtcctggcaccacagtacattctggacaggcccccagttcctctgtcaaggcagctgagaagcccctcaccttgcagggagggacgttgaaggctcgtgtcctcagatccaccctctgaaaggagtcaatgaagggcaagagcagaaccatgccaggtccctggggggtgcggatccggcccaggcggaacacaatcatccgctcgtaggtgggcacaatcttcagggcaaaccagccagaaatggggaaggtgaccaacagcagcaagaaccccaggaaactgatgaggccatgacagaggcaggagggccagctctggggtacatcggcccctgtccccacgccgccccgctccggggacaagcagcccttctgcgagcccagaaagccgaagctcgactgctggaagcggtcaaaatcacccaggggcagcgcccggtacccagacctgccgagcatggcttttgacaggagacacgccccgcgcctccgcgcggcgccctccctggccagtgggccctacgcggcccc

SEQ ID NO: 16605 - RNA, 2413 nt, Homo sapiens
  source 1..2413: mol_type = other RNA
gtgggctgggctgggctgggcctggggccagacctcaatgactgtttccttcccgtcagcgagcggagaagcagtgacagagtgtaccaggaggggaagctgacggtggccccaactcctctcttgaatgggatatgaccaccccacctgcccctcagtgtttgcaggacactctggcacactcatgccttcctttcctggtgaacctgtatcccactacaaagaggaacagaactccccacccagccccacccttgcttccaggggctttgagacactcaggagaaggagcttcaaatattgtgagggtctgtctgtgtcagccaccaggatgtcaatccctgcctgggctggcagcatggaccttgtggaccctcctagcccaccccatgcccccaggagccccgcttggcttcttctcttttatacattgtaaacaccacatttatttgtctgaggcttgcaaacctctggtaagaagcacagaacgcagggctctccttcatgctgccctgggccccagctcgccaggcatgcaggacagagctggcagatgagtcagaaatctttgggagcagcgccagggaagcagcaggccctgctccttcccatgcccaatcccgccagcacgggcctggactgcagccaggaaggtgggccagccaggatccccaggtaacttcgccacagggacctcttcttggagctgccttcccttccctccccatccctctccaatccccgcagagcttagagcctgggccacatgcttggtccctcacacaaggaccaaaccagctgctgtcaggctgtttctgtgggtcctgtctctccagtcaggaagccagcagggcagggcaggcctggctctcctcctggaatcacaccgtgcacccagctcagcgctgggcactcagctggggaccgggatggacaaagccttgtccagagaaccactgtaggggagacgtgcatggcagccggactcagcctcctgcagcctccattcatgggctcttggctgggcctgaaatttgttagggcctcaactctctgtggtgcagatgaacacctcctcctccaagaggcccctcaggcttggtgccaggcttgggactgggctctggaaagtcagccaaggctgctacttcaaggccctgaggacagcctccagcttcatggccatagccaggtcgcccttcaccttcagccgtccactcatgtaggcccccaggggccgcagctctctgcatagcagggcccgcaggtctgcctcggccatctccaccaccacatcagggatgccatcaggcaccccgtgtcccactcttcctcgtcctgtagtgaggtccaggaagtaggcgctttgggtgccgctgggcaggacgacattgaactggtagcaggccccgacttggctgaccagggcctcagacaggaagggctgtagagcagtcagtagcccctccgccagaggctgcttcggactggacctggcaccaacttgaggggcaggtggctcaacttcactcaccatctccacggtgtctgctggccccggggacggggcacctcctgccattgagttcatgcttcctcccaggaagtgcagggccagctgctggagggtgctgtccaggttgggcccagctgggctgtcctggggcggctggagcacggcctccactgccagctccacgcggtctacctccagcccccaggccctggtcacatcgttgatctccagcagaagctggtcgctgatcttgagcttctccatctggatctcccgcagcggcctcttgagcagggccttggtcatggcgttctgggctgtcatgcgtgtggctgtgttcaggtctttcacagtcatcaccgacagcaccgggtcccagatgcgaaactggacatcggctcccacggacagcacagccccgtccttagaggccagcttgcagggagggacgttgaaggctcgtgtcctcagatccaccctctgaaaggagtcaatgaagggcaagagcagaaccatgccaggtccctggggggtgcggatccggcccaggcggaacacaatcatccgctcgtaggtgggcacaatcttcagggcaaaccagccagaaatggggaaggtgaccaacagcagcaagaaccccaggaaactgatgaggccatgacagaggcaggagggccagctctggggtacatcggcccctgtccccacgccgccccgctccggggacaagcagcccttctgcgagcccagaaagccgaagctcgactgctggaagcggtcaaaatcacccaggggcagcgcccggtacccagacctgccgagcatggcttttgacaggagacacgccccgcgcctccgcgcggcgccctccctggccagtgggccctacgcggcccc

SEQ ID NO: 16606 - RNA, 2291 nt, Homo sapiens
  source 1..2291: mol_type = other RNA
gtgggctgggctgggctgggcctggggccagacctcaatgactgtttccttcccgtcagcgagcggagaagcagtgacagagtgtaccaggaggggaagctgacggtggccccaactcctctcttgaatgggatatgaccaccccacctgcccctcagtgtttgcaggacactctggcacactcatgccttcctttcctggtgaacctgtatcccactacaaagaggaacagaactccccacccagccccacccttgcttccaggggctttgagacactcaggagaaggagcttcaaatattgtgagggtctgtctgtgtcagccaccaggatgtcaatccctgcctgggctggcagcatggaccttgtggaccctcctagcccaccccatgcccccaggagccccgcttggcttcttctcttttatacattgtaaacaccacatttatttgtctgaggcttgcaaacctctggtaagaagcacagaacgcagggctctccttcatgctgccctgggccccagctcgccaggcatgcaggacagagctggcagatgagtcagaaatctttgggagcagcgccagggaagcagcaggccctgctccttcccatgcccaatcccgccagcacgggcctggactgcagccaggaaggtgggccagccaggatccccaggtaacttcgccacagggacctcttcttggagctgccttcccttccctccccatccctctccaatccccgcagagcttagagcctgggccacatgcttggtccctcacacaaggaccaaaccagctgctgtcaggctgtttctgtgggtcctgtctctccagtcaggaagccagcagggcagggcaggcctggctctcctcctggaatcacaccgtgcacccagctcagcgctgggcactcagctggggaccgggatggacaaagccttgtccagagaaccactgtaggggagacgtgcatggcagccggactcagcctcctgcagcctccattcatgggctcttggctgggcctgaaatttgttagggcctcaactctctgtggtgcagatgaacacctcctcctccaagaggcccctcaggcttggtgccaggcttgggactgggctctggaaagtcagccaaggctgctacttcaaggccctgaggacagcctccagcttcatggccatagccaggtcgcccttcaccttcagccgtccactcatgtaggcccccaggggccgcagctctctgcatagcagggcccgcaggtctgcctcggccatctccaccaccacatcagggatgccatcaggcaccccgtgtcccactcttcctcgtcctgtagtgaggtccaggaagtaggcgctttgggtgccgctgggcaggacgacattgaactggtagcaggccccgacttggctgaccagggcctcagacaggaagggctgtagagcagtcagtagcccctccgccagaggctgcttcggactggacctggcaccaacttgaggggcaggtggctcaacttcactcaccatctccacggtgtctgctggccccggggacggggcacctcctgccattgagttcatgcttcctcccaggaagtgcagggccagctgctggagggtgctgtccaggttgggcccagctgggctgtcctggggcggctggagcacggcctccactgccagctccacgcggtctacctccagcccccaggccctggtcacatcgttgatctccagcagaagctggtcgctgatcttgagcttctccatctggatctcccgcagcggcctcttgagcagggccttggtcatggcgttctgggctgtcatgcgtgtggctgtgttcaggtctttcacagtcatcaccgacagcaccgggtcccagatgcgaaactggacatcggctcccacggacagcacagccccgtccttagaggccagcttgcagggagggacgttgaaggctcgtgtcctcagatccaccctctgaaaggagtcaatgaagggcaagagcagaaccatgccaggtccctggggggtgcggatccggcccaggcggaacacaatcatccgctcgtaggtgggcacaatcttcagggcaaaccagccagaaatggggaaggtgaccaacagcagcaagaaccccaggaaactgatgaggccatgacagaggcaggagggccagctctggggtacatctgccgagcatggcttttgacaggagacacgccccgcgcctccgcgcggcgccctccctggccagtgggccctacgcggcccc

SEQ ID NO: 16607 - RNA, 2544 nt, Homo sapiens
  source 1..2544: mol_type = other RNA
gtgggctgggctgggctgggcctggggccagacctcaatgactgtttccttcccgtcagcgagcggagaagcagtgacagagtgtaccaggaggggaagctgacggtggccccaactcctctcttgaatgggatatgaccaccccacctgcccctcagtgtttgcaggacactctggcacactcatgccttcctttcctggtgaacctgtatcccactacaaagaggaacagaactccccacccagccccacccttgcttccaggggctttgagacactcaggagaaggagcttcaaatattgtgagggtctgtctgtgtcagccaccaggatgtcaatccctgcctgggctggcagcatggaccttgtggaccctcctagcccaccccatgcccccaggagccccgcttggcttcttctcttttatacattgtaaacaccacatttatttgtctgaggcttgcaaacctctggtaagaagcacagaacgcagggctctccttcatgctgccctgggccccagctcgccaggcatgcaggacagagctggcagatgagtcagaaatctttgggagcagcgccagggaagcagcaggccctgctccttcccatgcccaatcccgccagcacgggcctggactgcagccaggaaggtgggccagccaggatccccaggtaacttcgccacagggacctcttcttggagctgccttcccttccctccccatccctctccaatccccgcagagcttagagcctgggccacatgcttggtccctcacacaaggaccaaaccagctgctgtcaggctgtttctgtgggtcctgtctctccagtcaggaagccagcagggcagggcaggcctggctctcctcctggaatcacaccgtgcacccagctcagcgctgggcactcagctggggaccgggatggacaaagccttgtccagagaaccactgtaggggagacgtgcatggcagccggactcagcctcctgcagcctccattcatgggctcttggctgggcctgaaatttgttagggcctcaactctctgtggtgcagatgaacacctcctcctccaagaggcccctcaggcttggtgccaggcttgggactgggctctggaaagtcagccaaggctgctacttcaaggccctgaggacagcctccagcttcatggccatagccaggtcgcccttcaccttcagccgtccactcatgtaggcccccaggggccgcagctctctgcatagcagggcccgcaggtctgcctcggccatctccaccaccacatcagggatgccatcaggcaccccgtgtcccactcttcctcgtcctgtagtgaggtccaggaagtaggcgctttgggtgccgctgggcaggacgacattgaactggtagcaggccccgacttggctgaccagggcctcagacaggaagggctgtagagcagtcagtagcccctccgccagaggctgcttcggactggacctggcaccaacttgaggggcaggtggctcaacttcactcaccatctccacggtgtctgctggccccggggacggggcacctcctgccattgagttcatgcttcctcccaggaagtgcagggccagctgctggagggtgctgtccaggttgggcccagctgggctgtcctggggcggctggagcacggcctccactgccagctccacgcggtctacctccagcccccaggccctggtcacatcgttgatctccagcagaagctggtcgctgatcttgagcttctccatctggatctcccgcagcggcctcttgagcagggccttggtcatggcgttctgggctgtcatgcgtgtggctgtgttcaggtctttcacagtcatcaccgacagcaccgggtcccagatgcgaaactggacatcggctcccacggacagcacagccccgtccttagaggccagcttgcagggagggacgttgaaggctcgtgtcctcagatccaccctctgaaaggagtcaatgaagggcaagagcagaaccatgccaggtccctggggggtgcggatccggcccaggcggaacacaatcatccgctcgtaggtgggcacaatcttcagggcaaaccagccagaaatggggaaggtgaccaacagcagcaagaaccccaggaaactgatgaggccatgacagaggcaggagggccagctctggggtacatctggcatggagccaggagcacctgggcatctgtaaacatgcactgaatactgctggcaaaacacattcctcctataccatcagccccagaagtgtgctttccaggagtccttatgaagatgatgccttagccggcccctgtccccacgccgccccgctccggggacaagcagcccttctgcgagcccagaaagccgaagctcgactgctggaagcggtcaaaatcacccaggggcagcgcccggtacccagacctgccgagcatggcttttgacaggagacacgccccgcgcctccgcgcggcgccctccctggccagtgggccctacgcggcccc

SEQ ID NO: 16608 - RNA, 2260 nt, Homo sapiens
  source 1..2260: mol_type = other RNA
gtgggctgggctgggctgggcctggggccagacctcaatgactgtttccttcccgtcagcgagcggagaagcagtgacagagtgtaccaggaggggaagctgacggtggccccaactcctctcttgaatgggatatgaccaccccacctgcccctcagtgtttgcaggacactctggcacactcatgccttcctttcctggtgaacctgtatcccactacaaagaggaacagaactccccacccagccccacccttgcttccaggggctttgagacactcaggagaaggagcttcaaatattgtgagggtctgtctgtgtcagccaccaggatgtcaatccctgcctgggctggcagcatggaccttgtggaccctcctagcccaccccatgcccccaggagccccgcttggcttcttctcttttatacattgtaaacaccacatttatttgtctgaggcttgcaaacctctggtaagaagcacagaacgcagggctctccttcatgctgccctgggccccagctcgccaggcatgcaggacagagctggcagatgagtcagaaatctttgggagcagcgccagggaagcagcaggccctgctccttcccatgcccaatcccgccagcacgggcctggactgcagccaggaaggtgggccagccaggatccccaggtaacttcgccacagggacctcttcttggagctgccttcccttccctccccatccctctccaatccccgcagagcttagagcctgggccacatgcttggtccctcacacaaggaccaaaccagctgctgtcaggctgtttctgtgggtcctgtctctccagtcaggaagccagcagggcagggcaggcctggctctcctcctggaatcacaccgtgcacccagctcagcgctgggcactcagctggggaccgggatggacaaagccttgtccagagaaccactgtaggggagacgtgcatggcagccggactcagcctcctgcagcctccattcatgggctcttggctgggcctgaaatttgttagggcctcaactctctgtggtgcagatgaacacctcctcctccaagaggcccctcaggcttggtgccaggcttgggactgggctctggaaagtcagccaaggctgctacttcaaggccctgaggacagcctccagcttcatggccatagccaggtcgcccttcaccttcagccgtccactcatgtaggcccccaggggccgcagctctctgcatagcagggcccgcaggtctgcctcggccatctccaccaccacatcagggatgccatcaggcaccccgtgtcccactcttcctcgtcctgtagtgaggtccaggaagtaggcgctttgggtgccgctgggcaggacgacattgaactggtagcaggccccgacttggctgaccagggcctcagacaggaagggctgtagagcagtcagtagcccctccgccagaggctgcttcggactggacctggcaccaacttgaggggcaggtggctcaacttcactcaccatctccacggtgtctggccccggggacggggcacctcctgccattgagttcatgcttcctcccaggaagtgcagggccagctgctggagggtgctgtccaggttgggcccagctgggctgtcctggggcggctggagcacggcctccactgccagctccacgcggtctacctccagcccccaggccctggtcacatcgttgatctccagcagaagctggtcgctgatcttgagcttctccatctggatctcccgcagcggcctcttgagcagggccttggtcatggcgttctgggctgtcatgcgtgtggctgtgttcaggtctttcacagtcatcaccgacagcaccgggtcccagatgcgaaactggacatcggctcccacggacagcacagccccgtccttagaggccagcttcagggcaaaccagccagaaatggggaaggtgaccaacagcagcaagaaccccaggaaactgatgaggccatgacagaggcaggagggccagctctggggtacatcggcccctgtccccacgccgccccgctccggggacaagcagcccttctgcgagcccagaaagccgaagctcgactgctggaagcggtcaaaatcacccaggggcagcgcccggtacccagacctgccgagcatggcttttgacaggagacacgccccgcgcctccgcgcggcgccctccctggccagtgggccctacgcggcccc

SEQ ID NO: 16609 - RNA, 2410 nt, Homo sapiens
  source 1..2410: mol_type = other RNA
gtgggctgggctgggctgggcctggggccagacctcaatgactgtttccttcccgtcagcgagcggagaagcagtgacagagtgtaccaggaggggaagctgacggtggccccaactcctctcttgaatgggatatgaccaccccacctgcccctcagtgtttgcaggacactctggcacactcatgccttcctttcctggtgaacctgtatcccactacaaagaggaacagaactccccacccagccccacccttgcttccaggggctttgagacactcaggagaaggagcttcaaatattgtgagggtctgtctgtgtcagccaccaggatgtcaatccctgcctgggctggcagcatggaccttgtggaccctcctagcccaccccatgcccccaggagccccgcttggcttcttctcttttatacattgtaaacaccacatttatttgtctgaggcttgcaaacctctggtaagaagcacagaacgcagggctctccttcatgctgccctgggccccagctcgccaggcatgcaggacagagctggcagatgagtcagaaatctttgggagcagcgccagggaagcagcaggccctgctccttcccatgcccaatcccgccagcacgggcctggactgcagccaggaaggtgggccagccaggatccccaggtaacttcgccacagggacctcttcttggagctgccttcccttccctccccatccctctccaatccccgcagagcttagagcctgggccacatgcttggtccctcacacaaggaccaaaccagctgctgtcaggctgtttctgtgggtcctgtctctccagtcaggaagccagcagggcagggcaggcctggctctcctcctggaatcacaccgtgcacccagctcagcgctgggcactcagctggggaccgggatggacaaagccttgtccagagaaccactgtaggggagacgtgcatggcagccggactcagcctcctgcagcctccattcatgggctcttggctgggcctgaaatttgttagggcctcaactctctgtggtgcagatgaacacctcctcctccaagaggcccctcaggcttggtgccaggcttgggactgggctctggaaagtcagccaaggctgctacttcaaggccctgaggacagcctccagcttcatggccatagccaggtcgcccttcaccttcagccgtccactcatgtaggcccccaggggccgcagctctctgcatagcagggcccgcaggtctgcctcggccatctccaccaccacatcagggatgccatcaggcaccccgtgtcccactcttcctcgtcctgtagtgaggtccaggaagtaggcgctttgggtgccgctgggcaggacgacattgaactggtagcaggccccgacttggctgaccagggcctcagacaggaagggctgtagagcagtcagtagcccctccgccagaggctgcttcggactggacctggcaccaacttgaggggcaggtggctcaacttcactcaccatctccacggtgtctggccccggggacggggcacctcctgccattgagttcatgcttcctcccaggaagtgcagggccagctgctggagggtgctgtccaggttgggcccagctgggctgtcctggggcggctggagcacggcctccactgccagctccacgcggtctacctccagcccccaggccctggtcacatcgttgatctccagcagaagctggtcgctgatcttgagcttctccatctggatctcccgcagcggcctcttgagcagggccttggtcatggcgttctgggctgtcatgcgtgtggctgtgttcaggtctttcacagtcatcaccgacagcaccgggtcccagatgcgaaactggacatcggctcccacggacagcacagccccgtccttagaggccagcttgcagggagggacgttgaaggctcgtgtcctcagatccaccctctgaaaggagtcaatgaagggcaagagcagaaccatgccaggtccctggggggtgcggatccggcccaggcggaacacaatcatccgctcgtaggtgggcacaatcttcagggcaaaccagccagaaatggggaaggtgaccaacagcagcaagaaccccaggaaactgatgaggccatgacagaggcaggagggccagctctggggtacatcggcccctgtccccacgccgccccgctccggggacaagcagcccttctgcgagcccagaaagccgaagctcgactgctggaagcggtcaaaatcacccaggggcagcgcccggtacccagacctgccgagcatggcttttgacaggagacacgccccgcgcctccgcgcggcgccctccctggccagtgggccctacgcggcccc

SEQ ID NO: 16610 - RNA, 446 nt, Homo sapiens
  source 1..446: mol_type = other RNA
gtggggccaggcggtgggcacacacgcgcatgctggggggcgggtagcagcgagcgttgtcctcgacgggccccgtgacatgggcccgcagctcagtcaggttgggggccagcttaaagactcggttcactgcgcccacgaacacctccccagtcacccggtgcacagccaggtgggtaagcgtggtgtctgtcaccacgaaggcacggaagggcctgttgcccagggccccccccacggcaaggaagagcagcaggaggaggcagacagagggcatggccggcagccgcgcctggggacaggcctgtccctccgctggctccgggtggccgccctctggccacgtggacgcgcccccgagccccaccgcggccccgctcgcacgtccccacggcctcgccccgcgccccgggccccaagcgcgcagccgccgccgccgccgccca

SEQ ID NO: 16611 - RNA, 452 nt, Homo sapiens
  source 1..452: mol_type = other RNA
gtggggccaggcggtgggcacacacgcgcatgctggggggcgggtagcagcgagcgttgtcctcgacgggccccgtgacatgggcccgcagctcagtcaggttgggggccagcttaaagactcggttcactgcgcccacgaacacctccccagtcacccggtgcacagccaggtgggtaagcgtggtgtctgtcaccacgaaggcacggaagggcctgttgcccagggccccccccacggcaaggaagagcagcaggaggaggcagacagagggcatggccggcagccgcgcctggggacaggcctgtccctccgctggctccgggtggccgccctctggccacgtggacgcgcccccgagccccaccgcggccccgctcgcacgtccccacggcctcgccccgcgccccgggccccaagcgcgcagccgccgccgccgccgcccacacact

SEQ ID NO: 16612 - RNA, 124 nt, Homo sapiens
  source 1..124: mol_type = other RNA
gtggggccaggcggtgggcacacacgcgcatgctgtccctccgctggctccgggtggccgccctctggccacgtggacgcgcccccgagccccaccgcggccccgctcgcacgtccccacggcc

SEQ ID NO: 16613 - RNA, 2978 nt, Homo sapiens
  source 1..2978: mol_type = other RNA
gtgggggagaggctgtcagattctgagctccagaacctcaggtgtagcactgggattgggggtgggggctcaggaaccacctaggggagaagacagggtgggaagaaacaggaaggaaggtccccaaaattatgtttgtttgcagaggccagccaggctccaggggagtgtggactcagtcgaaccatagggccccaggaccactagcttctggccagcagtcatgccctccacagagctgggtccgtggaaattgcatgtaggagacacaccagactcccaggacagagcccttttgggatggccagcactacccagcctccactggtgagggaggtcaggggctgtgtgacctttgcttctgggactgatggtttattgagctggagagtgtgcccagcagtgttctccagccctcaggaacttctaatgtggctctgggttcctggagtgggtgggtcgaagctccactcggggaagaaacttccaagctgcctgcaggtgctggaggtccggtgattcactggctctgcccctgcagttcaagttcctggagtggctgtcagtggccacctgtctttaaatctgttcattttaggagctacctctcaccagaggcaggatcttggcatctggacttgatctgcttgggggtcaggcgagactgctggcagaggcttctcagggtggctgctgggctcatgagagttctcagggtccaggggccagggctgtccagtggctgtggggcccaactccatggggtgaacgccgcccagggggtggtccctgtgtgggccatctttggggccactgcacgcagggtcccttctgcagccccagctgcatcgctgcagatgggctcctgggagtcggtagcaacaccaggccaggccggcccctgggagcagaggcagcaggacgctgaggagcatggccagcaggaaggtgtcatggttttcagcctgcacagggccactgtccatgctgccaccaaagcctggcttgtcacagaagggtggagcccagcctggagcacagtggcagttatggttgctattgcaaaccattctaggtccacactgggtgcctggctctaccaggcccaggccaagcaggtccagctgggcactggggagtgccaaggctccccgacaagtcacttcctggccatctaggtgaacggtagagtccactggcaccatgtgcggtgcgagcaggctgggctttccaccctggcactgcagcttcccacacagggcatccctccctgcacagggcaggaagtggccctcgctgtcctggccgcagtttccatgagcatctcccgcagagttcaccacctggaaacaggcctcgggagctgggtgggagccaggcccccagagctgctggcactgctgctccagcgtgggacatgcgccatcccagcagtagccactgcccctggcacagggtgagccgtccagtaggtaaacgtctgggggacagtgggaggaggtgcccgtgcaaaactcagggaggtcacagtcacccatggcctggcggcacagcgctccagccggcttcagcaggcagcgcacgcagcagtccccgtgggcgcactgggcccccgggcgcagcgagcagttgtgagcaaagcagcagaggtcgcggcactcctggccagggccgcagtcacactcctcgcccgcttccacgaagccgttcccgcagagcgccggcggcaccgggagtccggggtccggggcattggagaggcaagcgccgccccccttgcggaagaaggcgcgcagctggcggcggctgcaggcgctgaacacgcgcggaaacgggtgcccggtggccgcagccatgacgcagcctccggactcggccgcagcctccacgcagcagccgtcggggtcgtggctgaggccgaggctgtggccgatctcatgggccatggtggctgcggcgccgatggggagctccgagtggtccgtgctcacgcctcccgagctctcggcgcggcacatgccctcgacgggcgccaggcccactgtggcgccctggaaggcgcggcccgtgagcagctgcgcggagtcgtggggccgctgcgcccacagcccccggcgccactgcaggaaggcccagagcgtggcgttggcgtcctgcgtgacgcggctgcggtcccgctcggtccacacctccaggccggtcagcgccacctgaatgtccagagtcctgagaagctggtccacgtagttggcgacttccaggagacgctgtttggtgtggttcaagtttcggtgccgagtcaagaacagggtgtggtctgccacaatgtacagttccaggtacttccgggtcctgcgcgcttctcgcctgcccctgctctggggaccaccaggaaggctggtcatgcccgctttgttcccaggatccctgtggccacaggttcctttccaggtgagcagctgctccatccgaaagatctcgtgggttgagaagtccttggagccccggggtggccagggacgcagataatagctggcattcctgctgagggtgatcaggccactcatcccagagcaggtgcagaggactacccaggagtcggggaagccccttactcgcccttggtagtggcaatgatccgtgtggttgggggccagcaccactggctgcccatctgggccgtagtgggtttctatgtatcctggggccagcagcctgtggttcttctccagctcaagcaggagctcctggccttcagcctccagggccaccagccccatgtctggcttcgagaccggctcctccaggctgacggtgcgccagggttgtccatccaggacccagtgcggggtgactggctgcccagggatatgtccttgaagcaccccggcgcctggcactggccagagcagcagcagtagtagcagcagcagcaacggggtcccccgagctctccggggcctccagcccatagctgt

SEQ ID NO: 16614 - RNA, 3056 nt, Homo sapiens
  source 1..3056: mol_type = other RNA
gtgggggagaggctgtcagattctgagctccagaacctcaggtgtagcactgggattgggggtgggggctcaggaaccacctaggggagaagacagggtgggaagaaacaggaaggaaggtccccaaaattatgtttgtttgcagaggccagccaggctccaggggagtgtggactcagtcgaaccatagggccccaggaccactagcttctggccagcagtcatgccctccacagagctgggtccgtggaaattgcatgtaggagacacaccagactcccaggacagagcccttttgggatggccagcactacccagcctccactggtgagggaggtcaggggctgtgtgacctttgcttctgggactgatggtttattgagctggagagtgtgcccagcagtgttctccagccctcaggaacttctaatgtggctctgggttcctggagtgggtgggtcgaagctccactcggggaagaaacttccaagctgcctgcaggtgctggaggtccggtgattcactggctctgcccctgcagttcaagttcctggagtggctgtcagtggccacctgtctttaaatctgttcattttaggagctacctctcaccagaggcaggatcttggcatctggacttgatctgcttgggggtcaggcgagactgctggcagaggcttctcagggtggctgctgggctcatgagagttctcagggtccaggggccagggctgtccagtggctgtggggcccaactccatggggtgaacgccgcccagggggtggtccctgtgtgggccatctttggggccactgcacgcagggtcccttctgcagccccagctgcatcgctgcagatgggctcctgggagtcggtagcaacaccaggccaggccggcccctgggagcagaggcagcaggacgctgaggagcatggccagcaggaaggtgtcatggttttcagcctgcacagggccactgtccatgctgccaccaaagcctggcttgtcacagaagggtggagcccagcctggagcacagtggcagttatggttgctattgcaaaccccgtggctgtggcaggcagtcaggcagcgctgaagctcctggaaggcattcttcctgcagcgcctgctctggcacaccattctaggtccacactgggtgcctggctctaccaggcccaggccaagcaggtccagctgggcactggggagtgccaaggctccccgacaagtcacttcctggccatctaggtgaacggtagagtccactggcaccatgtgcggtgcgagcaggctgggctttccaccctggcactgcagcttcccacacagggcatccctccctgcacagggcaggaagtggccctcgctgtcctggccgcagtttccatgagcatctcccgcagagttcaccacctggaaacaggcctcgggagctgggtgggagccaggcccccagagctgctggcactgctgctccagcgtgggacatgcgccatcccagcagtagccactgcccctggcacagggtgagccgtccagtaggtaaacgtctgggggacagtgggaggaggtgcccgtgcaaaactcagggaggtcacagtcacccatggcctggcggcacagcgctccagccggcttcagcaggcagcgcacgcagcagtccccgtgggcgcactgggcccccgggcgcagcgagcagttgtgagcaaagcagcagaggtcgcggcactcctggccagggccgcagtcacactcctcgcccgcttccacgaagccgttcccgcagagcgccggcggcaccgggagtccggggtccggggcattggagaggcaagcgccgccccccttgcggaagaaggcgcgcagctggcggcggctgcaggcgctgaacacgcgcggaaacgggtgcccggtggccgcagccatgacgcagcctccggactcggccgcagcctccacgcagcagccgtcggggtcgtggctgaggccgaggctgtggccgatctcatgggccatggtggctgcggcgccgatggggagctccgagtggtccgtgctcacgcctcccgagctctcggcgcggcacatgccctcgacgggcgccaggcccactgtggcgccctggaaggcgcggcccgtgagcagctgcgcggagtcgtggggccgctgcgcccacagcccccggcgccactgcaggaaggcccagagcgtggcgttggcgtcctgcgtgacgcggctgcggtcccgctcggtccacacctccaggccggtcagcgccacctgaatgtccagagtcctgagaagctggtccacgtagttggcgacttccaggagacgctgtttggtgtggttcaagtttcggtgccgagtcaagaacagggtgtggtctgccacaatgtacagttccaggtacttccgggtcctgcgcgcttctcgcctgcccctgctctggggaccaccaggaaggctggtcatgcccgctttgttcccaggatccctgtggccacaggttcctttccaggtgagcagctgctccatccgaaagatctcgtgggttgagaagtccttggagccccggggtggccagggacgcagataatagctggcattcctgctgagggtgatcaggccactcatcccagagcaggtgcagaggactacccaggagtcggggaagccccttactcgcccttggtagtggcaatgatccgtgtggttgggggccagcaccactggctgcccatctgggccgtagtgggtttctatgtatcctggggccagcagcctgtggttcttctccagctcaagcaggagctcctggccttcagcctccagggccaccagccccatgtctggcttcgagaccggctcctccaggctgacggtgcgccagggttgtccatccaggacccagtgcggggtgactggctgcccagggatatgtccttgaagcaccccggcgcctggcactggccagagcagcagcagtagtagcagcagcagcaacggggtcccccgagctctccggggcctccagcccatagctgt

SEQ ID NO: 16615 - RNA, 3053 nt, Homo sapiens
  source 1..3053: mol_type = other RNA
gtgggggagaggctgtcagattctgagctccagaacctcaggtgtagcactgggattgggggtgggggctcaggaaccacctaggggagaagacagggtgggaagaaacaggaaggaaggtccccaaaattatgtttgtttgcagaggccagccaggctccaggggagtgtggactcagtcgaaccatagggccccaggaccactagcttctggccagcagtcatgccctccacagagctgggtccgtggaaattgcatgtaggagacacaccagactcccaggacagagcccttttgggatggccagcactacccagcctccactggtgagggaggtcaggggctgtgtgacctttgcttctgggactgatggtttattgagctggagagtgtgcccagcagtgttctccagccctcaggaacttctaatgtggctctgggttcctggagtgggtgggtcgaagctccactcggggaagaaacttccaagctgcctgcaggtgctggaggtccggtgattcactggctctgcccctgcagttcaagttcctggagtggctgtcagtggccacctgtctttaaatctgttcattttaggagctacctctcaccagaggcaggatcttggcatctggacttgatctgcttgggggtcaggcgagactgctggcagaggcttctcagggtggctgctgggctcatgagagttctcagggtccaggggccagggctgtccagtggctgtggggcccaactccatggggtgaacgccgcccagggggtggtccctgtgtgggccatctttggggccactgcacgcagggtcccttctgcagccccagctgcatcgctgcagatgggctcctgggagtcggtagcaacaccaggccaggccggcccctgggagcagaggcagcaggacgctgaggagcatggccagcaggaaggtgtcatggttttcagcctgcacagggccactgtccatgctgccaccaaagcctggcttgtcacagaagggtggagcccagcctggagcacagtggcagttatggttgctattgcaaaccccgtggctgtggcaggcagtcaggcagcgctgaagctcctggaaggcattcttcctgcagcgcctgctctggcacaccattctaggtccacactgggtgcctggctctaccaggcccaggccaagcaggtccagctgggcactggggagtgccaaggctccccgacaagtcacttcctggccatctaggtgaacggtagagtccactggcaccatgtgcggtgcgagcaggctgggctttccaccctggcactgcagcttcccacacagggcatccctccctgcacagggcaggaagtggccctcgctgtcctggccgcagtttccatgagcatctcccgcagagttcaccacctggaaacaggcctcgggagctgggtgggagccaggcccccagagctgctggcactgctgctccagcgtgggacatgcgccatcccagcagtagccactgcccctggcacagggtgagccgtccagtaggtaaacgtctgggggacagtgggaggaggtgcccgtgcaaaactcagggaggtcacagtcacccatggcctggcggcacagcgctccagccggcttcagcaggcagcgcacgcagcagtccccgtgggcgcactgggcccccgggcgcagcgagcagttgtgagcaaagcagcagaggtcgcggcactcctggccagggccgcagtcacactcctcgcccgcttccacgaagccgttcccgcagagcgccggcggcaccgggagtccggggtccggggcattggagaggcaagcgccgccccccttgcggaagaaggcgcgcagctggcggcggctgcaggcgctgaacacgcgcggaaacgggtgcccggtggccgcagccatgacgcagcctccggactcggccgcagcctccacgcagcagccgtcggggtcgtggctgaggccgaggctgtggccgatctcatgggccatggtggctgcggcgccgatggggagctccgagtggtccgtgctcacgcctcccgagctctcggcgcggcacatgccctcgacgggcgccaggcccactgtggcgccctggaaggcgcggcccgtgagcagctgcgcggagtcgtggggccgctgcgcccacagcccccggcgccactgcaggaaggcccagagcgtggcgttggcgtcctgcgtgacgcggctgcggtcccgctcggtccacacctccaggccggtcagcgccacctgaatgtccagagtcctgagaagctggtccacgtagttggcgacttccaggagacgctgtttggtgtggttcaagtttcggtgccgagtcaagaacagggtgtggtctgccacaatgtacagttccaggtacttccgggtcctgcgcgcttctcgcctgcccctgctctggggaccaccaggaaggctggtcatgcccgctttgttcccaggatccctgtggccacaggttcctttccaggtgagcagctgctccatccgaaagatctcgtgggttgagaagtccttggagccccggggtggccagggacgcagataatagctggcattcctgctgagggtgatcaggccactcatcccagagcaggtgcagaggactacccaggagtcggggaagccccttactcgcccttggtagtggcaatgatccgtgtggttgggggccagcaccactggctgcccatctgggccgtagtgggtttctatgtatcctggggccagcagctggttcttctccagctcaagcaggagctcctggccttcagcctccagggccaccagccccatgtctggcttcgagaccggctcctccaggctgacggtgcgccagggttgtccatccaggacccagtgcggggtgactggctgcccagggatatgtccttgaagcaccccggcgcctggcactggccagagcagcagcagtagtagcagcagcagcaacggggtcccccgagctctccggggcctccagcccatagctgt

SEQ ID NO: 16616 - RNA, 3193 nt, Homo sapiens
  source 1..3193: mol_type = other RNA
gtgggggagaggctgtcagattctgagctccagaacctcaggtgtagcactgggattgggggtgggggctcaggaaccacctaggggagaagacagggtgggaagaaacaggaaggaaggtccccaaaattatgtttgtttgcagaggccagccaggctccaggggagtgtggactcagtcgaaccatagggccccaggaccactagcttctggccagcagtcatgccctccacagagctgggtccgtggaaattgcatgtaggagacacaccagactcccaggacagagcccttttgggatggccagcactacccagcctccactggtgagggaggtcaggggctgtgtgacctttgcttctgggactgatggtttattgagctggagagtgtgcccagcagtgttctccagccctcaggaacttctaatgtggctctgggttcctggagtgggtgggtcgaagctccactcggggaagaaacttccaagctgcctgcaggtgctggaggtccggtgattcactggctctgcccctgcagttcaagttcctggagtggctgtcagtggccacctgtctttaaatctgttcattttaggagctacctctcaccagaggcaggatcttggcatctggacttgatctgcttgggggtcaggcgagactgctggcagaggcttctcagggtggctgctgggctcatgagagttctcagggtccaggggccagggctgtccagtggctgtggggcccaactccatggggtgaacgccgcccagggggtggtccctgtgtgggccatctttggggccactgcacgcagggtcccttctgcagccccagctgcatcgctgcagatgggctcctgggagtcggtagcaacaccaggccaggccggcccctgggagcagaggcagcaggacgctgaggagcatggccagcaggaaggtgtcatggttttcagcctgcacagggccactgtccatgctgccaccaaagcctggcttgtcacagaagggtggagcccagcctggagcacagtggcagttatggttgctattgcaaaccccgtggctgtggcaggcagtcaggcagcgctgaagctcctggaaggcattcttcctgcagcgcctgctctggcacaccattctaggtccacactgggtgcctggctctaccaggcccaggccaagcaggtccagctgggcactggggagtgccaaggctccccgacaagtcacttcctggccatctaggtgaacggtagagtccactggcaccatgtgcggtgcgagcaggctgggctttccaccctggcactgcagcttcccacacagggcatccctccctgcacagggcaggaagtggccctcgctgtcctggccgcagtttccatgagcatctcccgcagagttcaccacctggaaacaggcctcgggagctgggtgggagccaggcccccagagctgctggcactgctgctccagcgtgggacatgcgccatcccagcagtagccactgcccctggcacagggtgagccgtccagtaggtaaacgtctgggggacagtgggaggaggtgcccgtgcaaaactcagggaggtcacagtcacccatggcctggcggcacagcgctccagccggcttcagcaggcagcgcacgcagcagtccccgtgggcgcactgggcccccgggcgcagcgagcagttgtgagcaaagcagcagaggtcgcggcactcctggccagggccgcagtcacactcctcgcccgcttccacgaagccgttcccgcagagcgccggcggcaccgggagtccggggtccggggcattggagaggcaagcgccgccccccttgcggaagaaggcgcgcagctggcggcggctgcaggcgctgaacacgcgcggaaacgggtgcccggtggccgcagccatgacgcagcctccggactcggccgcagcctccacgcagcagccgtcggggtcgtggctgaggccgaggctgtggccgatctcatgggccatggtggctgcggcgccgatggggagctccgagtggtccgtgctcacgcctcccgagctctcggcgcggcacatgccctcgacgggcgccaggcccactgtggcgccctggaaggcgcggcccgtgagcagctgcgcggagtcgtggggccgctgcgcccacagcccccggcgccactgcaggaaggcccagagcgtggcgttggcgtcctgcgtgacgcggctgcggtcccgctcggtccacacctccaggccggtcagcgccacctgaatgtccagagtcctgagaagctggtccacgtagttggcgacttccaggagacgctgtttggtgtggttcaagtttcggtgccgagtcaagaacagggtgtggtctgccacaatgtacagttccaggtacttccgggtcctgcgcgcttctcgcctgcccctgctctggggaccaccaggaaggctggtcatgcccgctttgttcccaggatccctgtggccacaggttcctttccaggtgagcagctgctccatccgaaagatctcgtgggttgagaagtccttggagccccggggtggccagggacgcagataatagctggcattcctgctgagggtgatcaggccactcatcccagagcaggtgcagaggactacccaggagtcggggaagccccttactcgcccttggtagtggcaatgatcctctggcggtgcatcccagagcccatggaagcatctcaccgtgtggttgggggccagcaccactggctgcccatctgggccgtagtgggtttctatgtatcctggggccagcagcctgtggttcttctccagctcaagcaggagctcctggccttcagcctccagggccaccagccccatgtctggcttcgagaccggctcctccaggctgacggtgcgccagggttgtccatccaggacccagtgcggggtgactggctgcccagggatatgtccttgaagcaccccggcgcctggcactggccagagcagcagcagtagtagcagcagcagcaacggggtcccccgagctctccggggcctccagcccatagctgtgagctcctcggcctctaggcagcggctcgcaactccggctccgcccaggctggattgcggccgacccgtgcccggtgcagcctcaggccgccgccttc

SEQ ID NO: 16617 - RNA, 3092 nt, Homo sapiens
  source 1..3092: mol_type = other RNA
gtgggggagaggctgtcagattctgagctccagaacctcaggtgtagcactgggattgggggtgggggctcaggaaccacctaggggagaagacagggtgggaagaaacaggaaggaaggtccccaaaattatgtttgtttgcagaggccagccaggctccaggggagtgtggactcagtcgaaccatagggccccaggaccactagcttctggccagcagtcatgccctccacagagctgggtccgtggaaattgcatgtaggagacacaccagactcccaggacagagcccttttgggatggccagcactacccagcctccactggtgagggaggtcaggggctgtgtgacctttgcttctgggactgatggtttattgagctggagagtgtgcccagcagtgttctccagccctcaggaacttctaatgtggctctgggttcctggagtgggtgggtcgaagctccactcggggaagaaacttccaagctgcctgcaggtgctggaggtccggtgattcactggctctgcccctgcagttcaagttcctggagtggctgtcagtggccacctgtctttaaatctgttcattttaggagctacctctcaccagaggcaggatcttggcatctggacttgatctgcttgggggtcaggcgagactgctggcagaggcttctcagggtggctgctgggctcatgagagttctcagggtccaggggccagggctgtccagtggctgtggggcccaactccatggggtgaacgccgcccagggggtggtccctgtgtgggccatctttggggccactgcacgcagggtcccttctgcagccccagctgcatcgctgcagatgggctcctgggagtcggtagcaacaccaggccaggccggcccctgggagcagaggcagcaggacgctgaggagcatggccagcaggaaggtgtcatggttttcagcctgcacagggccactgtccatgctgccaccaaagcctggcttgtcacagaagggtggagcccagcctggagcacagtggcagttatggttgctattgcaaaccccgtggctgtggcaggcagtcaggcagcgctgaagctcctggaaggcattcttcctgcagcgcctgctctggcacaccattctaggtccacactgggtgcctggctctaccaggcccaggccaagcaggtccagctgggcactggggagtgccaaggctccccgacaagtcacttcctggccatctaggtgaacggtagagtccactggcaccatgtgcggtgcgagcaggctgggctttccaccctggcactgcagcttcccacacagggcatccctccctgcacagggcaggaagtggccctcgctgtcctggccgcagtttccatgagcatctcccgcagagttcaccacctggaaacaggcctcgggagctgggtgggagccaggcccccagagctgctggcactgctgctccagcgtgggacatgcgccatcccagcagtagccactgcccctggcacagggtgagccgtccagtaggtaaacgtctgggggacagtgggaggaggtgcccgtgcaaaactcagggaggtcacagtcacccatggcctggcggcacagcgctccagccggcttcagcaggcagcgcacgcagcagtccccgtgggcgcactgggcccccgggcgcagcgagcagttgtgagcaaagcagcagaggtcgcggcactcctggccagggccgcagtcacactcctcgcccgcttccacgaagccgttcccgcagagcgccggcggcaccgggagtccggggtccggggcattggagaggcaagcgccgccccccttgcggaagaaggcgcgcagctggcggcggctgcaggcgctgaacacgcgcggaaacgggtgcccggtggccgcagccatgacgcagcctccggactcggccgcagcctccacgcagcagccgtcggggtcgtggctgaggccgaggctgtggccgatctcatgggccatggtggctgcggcgccgatggggagctccgagtggtccgtgctcacgcctcccgagctctcggcgcggcacatgccctcgacgggcgccaggcccactgtggcgccctggaaggcgcggcccgtgagcagctgcgcggagtcgtggggccgctgcgcccacagcccccggcgccactgcaggaaggcccagagcgtggcgttggcgtcctgcgtgacgcggctgcggtcccgctcggtccacacctccaggccggtcagcgccacctgaatgtccagagtcctgagaagctggtccacgtagttggcgacttccaggagacgctgtttggtgtggttcaagtttcggtgccgagtcaagaacagggtgtggtctgccacaatgtacagttccaggtacttccgggtcctgcgcgcttctcgcctgcccctgctctggggaccaccaggaaggctggtcatgcccgctttgttcccaggatccctgtggccacaggttcctttccaggtgagcagctgctccatccgaaagatctcgtgggttgagaagtccttggagccccggggtggccagggacgcagataatagctggcattcctgctgagggtgatcaggccactcatcccagagcaggtgcagaggactacccaggagtcggggaagccccttactcgcccttggtagtggcaatgatcctctggcggtgcatcccagagcccatggaagcatctcaccgtgtggttgggggccagcaccactggctgcccatctgggccgtagtgggtttctatgtatcctggggccagcagctggttcttctccagctcaagcaggagctcctggccttcagcctccagggccaccagccccatgtctggcttcgagaccggctcctccaggctgacggtgcgccagggttgtccatccaggacccagtgcggggtgactggctgcccagggatatgtccttgaagcaccccggcgcctggcactggccagagcagcagcagtagtagcagcagcagcaacggggtcccccgagctctccggggcctccagcccatagctgt

SEQ ID NO: 16618 - RNA, 3163 nt, Homo sapiens
  source 1..3163: mol_type = other RNA
gtgggggagaggctgtcagattctgagctccagaacctcaggtgtagcactgggattgggggtgggggctcaggaaccacctaggggagaagacagggtgggaagaaacaggaaggaaggtccccaaaattatgtttgtttgcagaggccagccaggctccaggggagtgtggactcagtcgaaccatagggccccaggaccactagcttctggccagcagtcatgccctccacagagctgggtccgtggaaattgcatgtaggagacacaccagactcccaggacagagcccttttgggatggccagcactacccagcctccactggtgagggaggtcaggggctgtgtgacctttgcttctgggactgatggtttattgagctggagagtgtgcccagcagtgttctccagccctcaggaacttctaatgtggctctgggttcctggagtgggtgggtcgaagctccactcggggaagaaacttccaagctgcctgcaggtgctggaggtccggtgattcactggctctgcccctgcagttcaagttcctggagtggctgtcagtggccacctgtctttaaatctgttcattttaggagctacctctcaccagaggcaggatcttggcatctggacttgatctgcttgggggtcaggcgagactgctggcagaggcttctcagggtggctgctgggctcatgagagttctcagggtccaggggccagggctgtccagtggctgtggggcccaactccatggggtgaacgccgcccagggggtggtccctgtgtgggccatctttggggccactgcacgcagggtcccttctgcagccccagctgcatcgctgcagatgggctcctgggagtcggtagcaacaccaggccaggccggcccctgggagcagaggcagcaggacgctgaggagcatggccagcaggaaggtgtcatggttttcagcctgcacagggccactgtccatgctgccaccaaagcctggcttgtcacagaagggtggagcccagcctggagcacagtggcagttatggttgctattgcaaaccccgtggctgtggcaggcagtcaggcagcgctgaagctcctggaaggcattcttcctgcagcgcctgctctggcacaccattctaggtccacactgggtgcctggctctaccaggcccaggccaagcaggtccagctgggcactggggagtgccaaggctccccgacaagtcacttcctggccatctaggtgaacggtagagtccactggcaccatgtgcggtgcgagcaggctgggctttccaccctggcactgcagcttcccacacagggcatccctccctgcacagggcaggaagtggccctcgctgtcctggccgcagtttccatgagcatctcccgcagagttcaccacctggaaacaggcctcgggagctgggtgggagccaggcccccagagctgctggcactgctgctccagcgtgggacatgcgccatcccagcagtagccactgcccctggcacagggtgagccgtccagtaggtaaacgtctgggggacagtgggaggaggtgcccgtgcaaaactcagggaggtcacagtcacccatggcctggcggcacagcgctccagccggcttcagcaggcagcgcacgcagcagtccccgtgggcgcactgggcccccgggcgcagcgagcagttgtgagcaaagcagcagaggtcgcggcactcctggccagggccgcagtcacactcctcgcccgcttccacgaagccgttcccgcagagcgccggcggcaccgggagtccggggtccggggcattggagaggcaagcgccgccccccttgcggaagaaggcgcgcagctggcggcggctgcaggcgctgaacacgcgcggaaacgggtgcccggtggccgcagccatgacgcagcctccggactcggccgcagcctccacgcagcagccgtcggggtcgtggctgaggccgaggctgtggccgatctcatgggccatggtggctgcggcgccgatggggagctccgagtggtcgcctcccgagctctcggcgcggcacatgccctcgacgggcgccaggcccactgtggcgccctggaaggcgcggcccctgggggcggagcgcggcgtgaccaggcggggccgggaggtgaggccgccccacccgggacccgcgtccgggtcagaggcacccacgtgagcagctgcgcggagtcgtggggccgctgcgcccacagcccccggcgccactgcaggaaggcccagagcgtggcgttggcgtcctgcgtgacgcggctgcggtcccgctcggtccacacctccaggccggtcagcgccacctgaatgtccagagtcctgagaagctggtccacgtagttggcgacttccaggagacgctgtttggtgtggttcaagtttcggtgccgagtcaagaacagggtgtggtctgccacaatgtacagttccaggtacttccgggtcctgcgcgcttctcgcctgcccctgctctggggaccaccaggaaggctggtcatgcccgctttgttcccaggatccctgtggccacaggttcctttccaggtgagcagctgctccatccgaaagatctcgtgggttgagaagtccttggagccccggggtggccagggacgcagataatagctggcattcctgctgagggtgatcaggccactcatcccagagcaggtgcagaggactacccaggagtcggggaagccccttactcgcccttggtagtggcaatgatccgtgtggttgggggccagcaccactggctgcccatctgggccgtagtgggtttctatgtatcctggggccagcagcctgtggttcttctccagctcaagcaggagctcctggccttcagcctccagggccaccagccccatgtctggcttcgagaccggctcctccaggctgacggtgcgccagggttgtccatccaggacccagtgcggggtgactggctgcccagggatatgtccttgaagcaccccggcgcctggcactggccagagcagcagcagtagtagcagcagcagcaacggggtcccccgagctctccggggcctccagcccatagctgtgagctcctcggcctctaggcagcggctcgc

SEQ ID NO: 16619 - RNA, 3184 nt, Homo sapiens
  source 1..3184: mol_type = other RNA
gtgggggagaggctgtcagattctgagctccagaacctcaggtgtagcactgggattgggggtgggggctcaggaaccacctaggggagaagacagggtgggaagaaacaggaaggaaggtccccaaaattatgtttgtttgcagaggccagccaggctccaggggagtgtggactcagtcgaaccatagggccccaggaccactagcttctggccagcagtcatgccctccacagagctgggtccgtggaaattgcatgtaggagacacaccagactcccaggacagagcccttttgggatggccagcactacccagcctccactggtgagggaggtcaggggctgtgtgacctttgcttctgggactgatggtttattgagctggagagtgtgcccagcagtgttctccagccctcaggaacttctaatgtggctctgggttcctggagtgggtgggtcgaagctccactcggggaagaaacttccaagctgcctgcaggtgctggaggtccggtgattcactggctctgcccctgcagttcaagttcctggagtggctgtcagtggccacctgtctttaaatctgttcattttaggagctacctctcaccagaggcaggatcttggcatctggacttgatctgcttgggggtcaggcgagactgctggcagaggcttctcagggtggctgctgggctcatgagagttctcagggtccaggggccagggctgtccagtggctgtggggcccaactccatggggtgaacgccgcccagggggtggtccctgtgtgggccatctttggggccactgcacgcagggtcccttctgcagccccagctgcatcgctgcagatgggctcctgggagtcggtagcaacaccaggccaggccggcccctgggagcagaggcagcaggacgctgaggagcatggccagcaggaaggtgtcatggttttcagcctgcacagggccactgtccatgctgccaccaaagcctggcttgtcacagaagggtggagcccagcctggagcacagtggcagttatggttgctattgcaaaccccgtggctgtggcaggcagtcaggcagcgctgaagctcctggaaggcattcttcctgcagcgcctgctctggcacaccattctaggtccacactgggtgcctggctctaccaggcccaggccaagcaggtccagctgggcactggggagtgccaaggctccccgacaagtcacttcctggccatctaggtgaacggtagagtccactggcaccatgtgcggtgcgagcaggctgggctttccaccctggcactgcagcttcccacacagggcatccctccctgcacagggcaggaagtggccctcgctgtcctggccgcagtttccatgagcatctcccgcagagttcaccacctggaaacaggcctcgggagctgggtgggagccaggcccccagagctgctggcactgctgctccagcgtgggacatgcgccatcccagcagtagccactgcccctggcacagggtgagccgtccagtaggtaaacgtctgggggacagtgggaggaggtgcccgtgcaaaactcagggaggtcacagtcacccatggcctggcggcacagcgctccagccggcttcagcaggcagcgcacgcagcagtccccgtgggcgcactgggcccccgggcgcagcgagcagttgtgagcaaagcagcagaggtcgcggcactcctggccagggccgcagtcacactcctcgcccgcttccacgaagccgttcccgcagagcgccggcggcaccgggagtccggggtccggggcattggagaggcaagcgccgccccccttgcggaagaaggcgcgcagctggcggcggctgcaggcgctgaacacgcgcggaaacgggtgcccggtggccgcagccatgacgcagcctccggactcggccgcagcctccacgcagcagccgtcggggtcgtggctgaggccgaggctgtggccgatctcatgggccatggtggctgcggcgccgatggggagctccgagtggtcgcctcccgagctctcggcgcggcacatgccctcgacgggcgccaggcccactgtggcgccctggaaggcgcggcccgtgagcagctgcgcggagtcgtggggccgctgcgcccacagcccccggcgccactgcaggaaggcccagagcgtggcgttggcgtcctgcgtgacgcggctgcggtcccgctcggtccacacctccaggccggtcagcgccacctgaatgtccagagtcctgagaagctggtccacgtagttggcgacttccaggagacgctgtttggtgtggttcaagtttcggtgccgagtcaagaacagggtgtggtctgccacaatgtacagttccaggtacttccgggtcctgcgcgcttctcgcctgcccctgctctggggaccaccaggaaggctggtcatgcccgctttgttcccaggatccctgtggccacaggttcctttccaggtgagcagctgctccatccgaaagatctcgtgggttgagaagtccttggagccccggggtggccagggacgcagataatagctggcattcctgctgagggtgatcaggccactcatcccagagcaggtgcagaggactacccaggagtcggggaagccccttactcgcccttggtagtggcaatgatcctctggcggtgcatcccagagcccatggaagcatctcaccgtgtggttgggggccagcaccactggctgcccatctgggccgtagtgggtttctatgtatcctggggccagcagcctgtggttcttctccagctcaagcaggagctcctggccttcagcctccagggccaccagccccatgtctggcttcgagaccggctcctccaggctgacggtgcgccagggttgtccatccaggacccagtgcggggtgactggctgcccagggatatgtccttgaagcaccccggcgcctggcactggccagagcagcagcagtagtagcagcagcagcaacggggtcccccgagctctccggggcctccagcccatagctgtgagctcctcggcctctaggcagcggctcgcaactccggctccgcccaggctggattgcggccgacccgtgcccggtgcagcctcaggccgccgccttc

SEQ ID NO: 16620 - RNA, 3158 nt, Homo sapiens
  source 1..3158: mol_type = other RNA
gtgggggagaggctgtcagattctgagctccagaacctcaggtgtagcactgggattgggggtgggggctcaggaaccacctaggggagaagacagggtgggaagaaacaggaaggaaggtccccaaaattatgtttgtttgcagaggccagccaggctccaggggagtgtggactcagtcgaaccatagggccccaggaccactagcttctggccagcagtcatgccctccacagagctgggtccgtggaaattgcatgtaggagacacaccagactcccaggacagagcccttttgggatggccagcactacccagcctccactggtgagggaggtcaggggctgtgtgacctttgcttctgggactgatggtttattgagctggagagtgtgcccagcagtgttctccagccctcaggaacttctaatgtggctctgggttcctggagtgggtgggtcgaagctccactcggggaagaaacttccaagctgcctgcaggtgctggaggtccggtgattcactggctctgcccctgcagttcaagttcctggagtggctgtcagtggccacctgtctttaaatctgttcattttaggagctacctctcaccagaggcaggatcttggcatctggacttgatcttgggggtcaggcgagactgctggcagaggcttctcagggtggctgctgggctcatgagagttctcagggtccaggggccagggctgtccagtggctgtggggcccaactccatggggtgaacgccgcccagggggtggtccctgtgtgggccatctttggggccactgcacgcagggtcccttctgcagccccagctgcatcgctgcagatgggctcctgggagtcggtagcaacaccaggccaggccggcccctgggagcagaggcagcaggacgctgaggagcatggccagcaggaaggtgtcatggttttcagcctgcacagggccactgtccatgctgccaccaaagcctggcttgtcacagaagggtggagcccagcctggagcacagtggcagttatggttgctattgcaaaccccgtggctgtggcaggcagtcaggcagcgctgaagctcctggaaggcattcttcctgcagcgcctgctctggcacaccattctaggtccacactgggtgcctggctctaccaggcccaggccaagcaggtccagctgggcactggggagtgccaaggctccccgacaagtcacttcctggccatctaggtgaacggtagagtccactggcaccatgtgcggtgcgagcaggctgggctttccaccctggcactgcagcttcccacacagggcatccctccctgcacagggcaggaagtggccctcgctgtcctggccgcagtttccatgagcatctcccgcagagttcaccaccaggcccccagagctgctggcactgctgctccagcgtgggacatgcgccatcccagcagtagccactgcccctggcacagggtgagccgtccagtaggtaaacgtctgggggacagtgggaggaggtgcccgtgcaaaactcagggaggtcacagtcacccatggcctggcggcacagcgctccagccggcttcagcaggcagcgcacgcagcagtccccgtgggcgcactgggcccccgggcgcagcgagcagttgtgagcaaagcagcagaggtcgcggcactcctggccagggccgcagtcacactcctcgcccgcttccacgaagccgttcccgcagagcgccggcggcaccgggagtccggggtccggggcattggagaggcaagcgccgccccccttgcggaagaaggcgcgcagctggcggcggctgcaggcgctgaacacgcgcggaaacgggtgcccggtggccgcagccatgacgcagcctccggactcggccgcagcctccacgcagcagccgtcggggtcgtggctgaggccgaggctgtggccgatctcatgggccatggtggctgcggcgccgatggggagctccgagtggtccgtgctcacgcctcccgagctctcggcgcggcacatgccctcgacgggcgccaggcccactgtggcgccctggaaggcgcggcccgtgagcagctgcgcggagtcgtggggccgctgcgcccacagcccccggcgccactgcaggaaggcccagagcgtggcgttggcgtcctgcgtgacgcggctgcggtcccgctcggtccacacctccaggccggtcagcgccacctgaatgtccagagtcctgagaagctggtccacgtagttggcgacttccaggagacgctgtttggtgtggttcaagtttcggtgccgagtcaagaacagggtgtggtctgccacaatgtacagttccaggtacttccgggtcctgcgcgcttctcgcctgcccctgctctggggaccaccaggaaggctggtcatgcccgctttgttcccaggatccctgtggccacaggttcctttccaggtgagcagctgctccatccgaaagatctcgtgggttgagaagtccttggagccccggggtggccagggacgcagataatagctggcattcctgctgagggtgatcaggccactcatcccagagcaggtgcagaggactacccaggagtcggggaagccccttactcgcccttggtagtggcaatgatcctctggcggtgcatcccagagcccatggaagcatctcaccgtgtggttgggggccagcaccactggctgcccatctgggccgtagtgggtttctatgtatcctggggccagcagcctgtggttcttctccagctcaagcaggagctcctggccttcagcctccagggccaccagccccatgtctggcttcgagaccggctcctccaggctgacggtgcgccagggttgtccatccaggacccagtgcggggtgactggctgcccagggatatgtccttgaagcaccccggcgcctggcactggccagagcagcagcagtagtagcagcagcagcaacggggtcccccgagctctccggggcctccagcccatagctgtgagctcctcggcctctaggcagcggctcgcaactccggctccgcccaggctggattgcggccgacccgtgcccggtgcagcctcaggccgccgccttc

SEQ ID NO: 16621 - RNA, 3053 nt, Homo sapiens
  source 1..3053: mol_type = other RNA
gtgggggagaggctgtcagattctgagctccagaacctcaggtgtagcactgggattgggggtgggggctcaggaaccacctaggggagaagacagggtgggaagaaacaggaaggaaggtccccaaaattatgtttgtttgcagaggccagccaggctccaggggagtgtggactcagtcgaaccatagggccccaggaccactagcttctggccagcagtcatgccctccacagagctgggtccgtggaaattgcatgtaggagacacaccagactcccaggacagagcccttttgggatggccagcactacccagcctccactggtgagggaggtcaggggctgtgtgacctttgcttctgggactgatggtttattgagctggagagtgtgcccagcagtgttctccagccctcaggaacttctaatgtggctctgggttcctggagtgggtgggtcgaagctccactcggggaagaaacttccaagctgcctgcaggtgctggaggtccggtgattcactggctctgcccctgcagttcaagttcctggagtggctgtcagtggccacctgtctttaaatctgttcattttaggagctacctctcaccagaggcaggatcttggcatctggacttgatcttgggggtcaggcgagactgctggcagaggcttctcagggtggctgctgggctcatgagagttctcagggtccaggggccagggctgtccagtggctgtggggcccaactccatggggtgaacgccgcccagggggtggtccctgtgtgggccatctttggggccactgcacgcagggtcccttctgcagccccagctgcatcgctgcagatgggctcctgggagtcggtagcaacaccaggccaggccggcccctgggagcagaggcagcaggacgctgaggagcatggccagcaggaaggtgtcatggttttcagcctgcacagggccactgtccatgctgccaccaaagcctggcttgtcacagaagggtggagcccagcctggagcacagtggcagttatggttgctattgcaaaccccgtggctgtggcaggcagtcaggcagcgctgaagctcctggaaggcattcttcctgcagcgcctgctctggcacaccattctaggtccacactgggtgcctggctctaccaggcccaggccaagcaggtccagctgggcactggggagtgccaaggctccccgacaagtcacttcctggccatctaggtgaacggtagagtccactggcaccatgtgcggtgcgagcaggctgggctttccaccctggcactgcagcttcccacacagggcatccctccctgcacagggcaggaagtggccctcgctgtcctggccgcagtttccatgagcatctcccgcagagttcaccacctggaaacaggcctcgggagctgggtgggagccaggcccccagagctgctggcactgctgctccagcgtgggacatgcgccatcccagcagtagccactgcccctggcacagggtgagccgtccagtaggtaaacgtctgggggacagtgggaggaggtgcccgtgcaaaactcagggaggtcacagtcacccatggcctggcggcacagcgctccagccggcttcagcaggcagcgcacgcagcagtccccgtgggcgcactgggcccccgggcgcagcgagcagttgtgagcaaagcagcagaggtcgcggcactcctggccagggccgcagtcacactcctcgcccgcttccacgaagccgttcccgcagagcgccggcggcaccgggagtccggggtccggggcattggagaggcaagcgccgccccccttgcggaagaaggcgcgcagctggcggcggctgcaggcgctgaacacgcgcggaaacgggtgcccggtggccgcagccatgacgcagcctccggactcggccgcagcctccacgcagcagccgtcggggtcgtggctgaggccgaggctgtggccgatctcatgggccatggtggctgcggcgccgatggggagctccgagtggtccgtgctcacgcctcccgagctctcggcgcggcacatgccctcgacgggcgccaggcccactgtggcgccctggaaggcgcggcccgtgagcagctgcgcggagtcgtggggccgctgcgcccacagcccccggcgccactgcaggaaggcccagagcgtggcgttggcgtcctgcgtgacgcggctgcggtcccgctcggtccacacctccaggccggtcagcgccacctgaatgtccagagtcctgagaagctggtccacgtagttggcgacttccaggagacgctgtttggtgtggttcaagtttcggtgccgagtcaagaacagggtgtggtctgccacaatgtacagttccaggtacttccgggtcctgcgcgcttctcgcctgcccctgctctggggaccaccaggaaggctggtcatgcccgctttgttcccaggatccctgtggccacaggttcctttccaggtgagcagctgctccatccgaaagatctcgtgggttgagaagtccttggagccccggggtggccagggacgcagataatagctggcattcctgctgagggtgatcaggccactcatcccagagcaggtgcagaggactacccaggagtcggggaagccccttactcgcccttggtagtggcaatgatccgtgtggttgggggccagcaccactggctgcccatctgggccgtagtgggtttctatgtatcctggggccagcagcctgtggttcttctccagctcaagcaggagctcctggccttcagcctccagggccaccagccccatgtctggcttcgagaccggctcctccaggctgacggtgcgccagggttgtccatccaggacccagtgcggggtgactggctgcccagggatatgtccttgaagcaccccggcgcctggcactggccagagcagcagcagtagtagcagcagcagcaacggggtcccccgagctctccggggcctccagcccatagctgt

SEQ ID NO: 16622 - RNA, 3267 nt, Homo sapiens
  source 1..3267: mol_type = other RNA
gtgggggagaggctgtcagattctgagctccagaacctcaggtgtagcactgggattgggggtgggggctcaggaaccacctaggggagaagacagggtgggaagaaacaggaaggaaggtccccaaaattatgtttgtttgcagaggccagccaggctccaggggagtgtggactcagtcgaaccatagggccccaggaccactagcttctggccagcagtcatgccctccacagagctgggtccgtggaaattgcatgtaggagacacaccagactcccaggacagagcccttttgggatggccagcactacccagcctccactggtgagggaggtcaggggctgtgtgacctttgcttctgggactgatggtttattgagctggagagtgtgcccagcagtgttctccagccctcaggaacttctaatgtggctctgggttcctggagtgggtgggtcgaagctccactcggggaagaaacttccaagctgcctgcaggtgctggaggtccggtgattcactggctctgcccctgcagttcaagttcctggagtggctgtcagtggccacctgtctttaaatctgttcattttaggagctacctctcaccagaggcaggatcttggcatctggacttgatcttgggggtcaggcgagactgctggcagaggcttctcagggtggctgctgggctcatgagagttctcagggtccaggggccagggctgtccagtggctgtggggcccaactccatggggtgaacgccgcccagggggtggtccctgtgtgggccatctttggggccactgcacgcagggtcccttctgcagccccagctgcatcgctgcagatgggctcctgggagtcggtagcaacaccaggccaggccggcccctgggagcagaggcagcaggacgctgaggagcatggccagcaggaaggtgtcatggttttcagcctgcacagggccactgtccatgctgccaccaaagcctggcttgtcacagaagggtggagcccagcctggagcacagtggcagttatggttgctattgcaaaccccgtggctgtggcaggcagtcaggcagcgctgaagctcctggaaggcattcttcctgcagcgcctgctctggcacaccattctaggtccacactgggtgcctggctctaccaggcccaggccaagcaggtccagctgggcactggggagtgccaaggctccccgacaagtcacttcctggccatctaggtgaacggtagagtccactggcaccatgtgcggtgcgagcaggctgggctttccaccctggcactgcagcttcccacacagggcatccctccctgcacagggcaggaagtggccctcgctgtcctggccgcagtttccatgagcatctcccgcagagttcaccacctggaaacaggcctcgggagctgggtgggagccaggcccccagagctgctggcactgctgctccagcgtgggacatgcgccatcccagcagtagccactgcccctggcacagggtgagccgtccagtaggtaaacgtctgggggacagtgggaggaggtgcccgtgcaaaactcagggaggtcacagtcacccatggcctggcggcacagcgctccagccggcttcagcaggcagcgcacgcagcagtccccgtgggcgcactgggcccccgggcgcagcgagcagttgtgagcaaagcagcagaggtcgcggcactcctggccagggccgcagtcacactcctcgcccgcttccacgaagccgttcccgcagagcgccggcggcaccgggagtccggggtccggggcattggagaggcaagcgccgccccccttgcggaagaaggcgcgcagctggcggcggctgcaggcgctgaacacgcgcggaaacgggtgcccggtggccgcagccatgacgcagcctccggactcggccgcagcctccacgcagcagccgtcggggtcgtggctgaggccgaggctgtggccgatctcatgggccatggtggctgcggcgccgatggggagctccgagtggtcctggggggccgtgggagggcggtcactgcggccgtagagcctcctgtctctccctcgcccccgcccgcggggctcaccgtgctcacgcctcccgagctctcggcgcggcacatgccctcgacgggcgccaggcccactgtggcgccctggaaggcgcggcccgtgagcagctgcgcggagtcgtggggccgctgcgcccacagcccccggcgccactgcaggaaggcccagagcgtggcgttggcgtcctgcgtgacgcggctgcggtcccgctcggtccacacctccaggccggtcagcgccacctgaatgtccagagtcctgagaagctggtccacgtagttggcgacttccaggagacgctgtttggtgtggttcaagtttcggtgccgagtcaagaacagggtgtggtctgccacaatgtacagttccaggtacttccgggtcctgcgcgcttctcgcctgcccctgctctggggaccaccaggaaggctggtcatgcccgctttgttcccaggatccctgtggccacaggttcctttccaggtgagcagctgctccatccgaaagatctcgtgggttgagaagtccttggagccccggggtggccagggacgcagataatagctggcattcctgctgagggtgatcaggccactcatcccagagcaggtgcagaggactacccaggagtcggggaagccccttactcgcccttggtagtggcaatgatcctctggcggtgcatcccagagcccatggaagcatctcaccgtgtggttgggggccagcaccactggctgcccatctgggccgtagtgggtttctatgtatcctggggccagcagcctgtggttcttctccagctcaagcaggagctcctggccttcagcctccagggccaccagccccatgtctggcttcgagaccggctcctccaggctgacggtgcgccagggttgtccatccaggacccagtgcggggtgactggctgcccagggatatgtccttgaagcaccccggcgcctggcactggccagagcagcagcagtagtagcagcagcagcaacggggtcccccgagctctccggggcctccagcccatagctgtgagctcctcggcctctaggcagcggctcgcaactccggctccgcccaggctggattgcggccgacccgtgcccggtgcagcctcaggccgccgccttc

SEQ ID NO: 16623 - RNA, 2292 nt, Homo sapiens
  source 1..2292: mol_type = other RNA
gtgtctgggcggacagctgcaaatgctacttggggaggggacacagggagccgacaggaagcggtcccgtccccaccaggcacctgctctggcccccgcccagcctggctttgccctcttgtgggtccgctgtccgttcctgatcttccccaggaactcgggccctccgtcagcactcgcacacagggacgcgttattttggtctttccatcttctgcttaatgggtgctccctctggtcaggacacatgtcccgcttattgtcgtgggcccagagccatccccacccgtttgctgtcctgctgggaactgtctggctctgggcgatatgaggagggactccagggagctgggaggggtctgagtgcagctgtggggaagcagaggccgagctgggctgtacagcatggaggtcccgcccaaccctccccttggggtgctgagcctgagcttggtagctggcagcatgggctcacctcctgcgccactgctgccaccagcgggacttaggccacgccacggcctttctgcctccatttccctgtctgtaaaatggagtgagagcagtgtctgtttcctcatctgtctcagtggcacttttggtagtgaggttggggtgagcctgctgcacgtggcaggtgctactcaaacagaagtgtcctggaggagggcagggggcgcggacactgggcaggggccgggcatttgctctggaggtgaacctggaggagggcagggggcgcggacgctgggcaggggccgggcatttgctctggaggtgaacctggaggagggccgggggcatggatgctgggcaggggccgggcacttgccctggaggtgaacctggaggagggctgggggcgcggacgctgggcaggggccgggcatttgctctggaggtgaacctggaggagggctgggggcatggatgctgggcaggggccgggcacttgccctggaggtgaacctggaggagggctgggggtgcggacgctgggcaggggccgggcatttgctctggaggtgaacctggaggagggctgggggcgcggacgctgggcaggggccgggcatttgctctggaggtgaacctggaggagggccgggggcatggatgctgggcaggggccgggcatttgctctggaggtgaacctggaggagggccgggggcatggatgctgggcaggggccgggcatttgctctggaggtgaacctggaggagggccgggggcgcggacgctgggcaggggccaggcatttgccctggaggtgaacctggaggagggccgggggcatggatgctgggcaggggccgggcatttgccctggaggtgaacctggaggagggccgggggcatggatgctgggcaggggccgggcatttgctctggaggtgaacctggaggagggccgggggcgcagacgctgggcaggggccgggcatttgctctggaggtgaacctggaggagggccgggggcatggatgctgggcaggggccgggcatttgctctggaggtgaacctggaggagggccgggggcgcggacgctgggcaggggccgggcatttgccctggaggtgaacctggaggagggccgggggcatggatgctgggcaggggccgggcatttgctctggaggtgaacctggaggagggccgggggcgcagacgctgggcaggggctgggcatttgctctggaggtgaacctggaggagggctgggggcatggatgctgggcaggggccgggcacttgccctggaggtgaacctggaggagggccgggggcatggatgctgggcaggggccgggcatttgctctggaggtgaacctggaggagggccgggggcatggatgctgggcaggggccgggcatttgccctggaggtgaacctggaggagggccgggggcgcggacgctgggcaggggccgggcatttgctctggaggtgaacctggaggagggccgggggatggatgctgggcaggggccgggcatttgccctggaggtgaacctggaggagggccgggggcgcggacgctgggcaggggccgggcatttgccctggaggtgaacctggaggagggccgggggcatggatgctgggcaggggccgggcatttgctctggaggtgaacctggaggagggccgggggcgcggacactgggcaggggccgggcacttgctctccgaagtgaacctggaggcctctgccacttggctctctgggtcgtgggtctggcaaggtcggggccaggaggccgccccgatggtgcctgttgc

SEQ ID NO: 16624 - RNA, 394 nt, Homo sapiens
  source 1..394: mol_type = other RNA
gtgtgaccaccgttcctgcaggcatgccaaaactttgttctcccctgtttgtctttttttgggggtggggggcgtaatttgagatcttcttcaagggggtttcctatttgcaaaaatctacaagaagtagcattaattttccggaagtaagtattgctaacacagagttaggactgtccagatcgtcagagtttcttggtgacgcttttacagtagccattctcaactcgggagattttcaaacatctgagtgtcttgcatttcgcgaccctgcagtactctgcttttgaaaagcaggaggcctactcctgctgctgtttatgtgactgcttcttagcacgctgctgttcctgctcccgcggctgctcgcctatgattgccttcttcacaatgc

SEQ ID NO: 16625 - RNA, 2032 nt, Homo sapiens
  source 1..2032: mol_type = other RNA
gtgtggaagatgggaggagaaaaggcagtctaggagaccaaaggaggcttctccagctccggaggctcaggcatgccagaaagaggcactctctggctccccttggacgacccactgtgtacaaagcacgccgtcattcgccatttttcagtatccttagggcagccctgagagtcacatcaagcgtgtgttatgattcccatttcatagatgagaaaactgaagctcagagacagaaaacgaggtcttcagactccaggtccagagtgtcatcccccaccaggtaggactgctttctttagggccctggactcaaaagagcatctgcagtcggccttttggaccacacaggaccagagagccttggtgaagagtaggtggttagggctgtcaggagcactttttggtgggccagaaaagcagggacaagcacaggtggaccaaggagctgcactccgaggccttgggccaaacctgagggtacctcctctgagttgcagccaaaagatctctggtccctcagaaatcccaacagcctctccatcttatgttaagctggagtttgctgctgtcctcgtctcctgctcatggacatctggagaatgtcagaaccagaggaaagaatgacagtcactggatgccagattcttcatcaatgctgcaagatgtctctggcctcacttagcatagcgacagagccttaagtgaacccatgcttcctggatccccacttagccttgtccttcctgctagtgggtgagcgagagagaggggccccctggctaagagacttggcaggggtgatgacaagatgctcagcaggatagagccatcagactgtggctgtcatcgggaaagacagagacgtttctgcttacaactttgaggcttccaaacttttcctggtacgagagagtgtttcttccaccttaaactacatgatggaaagatatgtgagaatagaaaaaaaaaagcgtgtgttgctatggaactgcaaatccctgatagaagtcttcctctgaaccacatcctgcatcgacgagaccacccagctagtcttagagcaagatggagtggccctctcaaatgctatcatttgctgttacctacattcctccaggccctatgtagcagcccctatcatagccatcaccctcaggatttgaatcaattccccagttagcacactaggggaaaacaaaggcctcatttgaagtctctcctgactgtattccttaggaagctgtcccacaatgcctcggtgagggctggcaggcgagctgactagcccctgccggacaactgtcaggttggttgaaggatattagagggaagttgatcatgtgtcaacgcttctcagcgcccactcacatcagggaagtgatacagctgtcactgtggccgacgaggcggctggcagaacaggccacgttcaccaacccagctgtccaattagatgcaagggcctgaccctcaggtgtgcgggaggcagggaagaagtgctgaggaggacaccactaccagcggtctctgaggctcctgggctgcctccctggctgcctgtgtcccactgaacagatcagggatgcagggacattcagtccagtgatgctggctccttcattctaaccttctcccatctgcatttctttatcctgtttcctcccttcctctctcctttcgtttcttccatcctcctttctcccttcctgtctcttggggtgggttatgtgatgagaatataaagaaaagttcccagaactcctctggggagacagtaggaaatatgtgagatttgattagacattgaaagaaaagccaaactgtggcagagaactctttagtgctttgttctcagtgcttttaagaatgctagtgtggtgtttgattaaagaacataatcaatttggaaacaatgctcagtgtgataacatgggggagtgttgttgaaaacactgctctttcttttttatccaattttccattagattttattttatttatttattttctatttaacttttttttttaa

SEQ ID NO: 16626 - RNA, 178 nt, Homo sapiens
  source 1..178: mol_type = other RNA
gtgtgtggaaatgcttctgcaaatccttcaggatagtctctgtcttttgtttcacacttctctgaaacacaaggattttgaacaggtaatgcaacgcctctgatgcctctatgctgatctcgtggttgcagcccatgacgaacaggccgaagatgctcatcagtttcccactcattga

SEQ ID NO: 16627 - RNA, 5199 nt, Homo sapiens
  source 1..5199: mol_type = other RNA
gtgttaattaaacctctatttacatgtgtatttgtaaaatacacttactacaactgctgctttaccttaaatcatagaaccattcagtactcacttcctcatgacatcaattatacctcctcactcataacacttcactaccatctaatcatgttttaaaattatacgaatctgtaccatcactgaccttctattcaaaaccattcttacaacataggaagtaaaaataaaattcattcaatgcactgaaagcaactaatgcatcagggatgacaacttggcaccaagaacctaactaaaaatggacaaagtatgttaaagtttggcttcctggagactttctcatcaggtctctggcccatttagaaaaagagagcttgaattttattatttcagttgctgggtaacatgcaatttccctgatatattgaactgatgcttttatttgatcacaggactcagccgttacaaaaataacaagtcattttctttaataaaaaataaaaggaagtatatggttgggtcctaagactctggagtaattgaatgtaagcttaaaacatactaaatattttccacttgggaaatctggagaaactaggtttctaggagcaactgcttcaatagttggtgtaaagaatatgtttcacttacacatgaaagtggacacatattattttgattctgcatacttttatgtctttcaattggcaatgcaagatgttccaggatatgaaactttcaccgacccttacattccatactcctcgccaatgtgttatgtcagaaattctgacattccaaattcatattggtctttattttcctaactgttgaagcagaagatagaacagcaatgcacccaagagtctggtaagctcaaatatgtggattttctgagtcttcagataaacaatgtagaaaataaattaaatggtaattttaaatgatttatccagcactaacatgtctccagtttcatctctagaaagccactgccaagtttttgcacaacctaatttatcaagctttgatagatgaaaaatcctctagtttcagtatctcttctcattattccatcatgtaatgttgcaattgattgattctcatttcatttcaagccctaggtcctcctcttcatacaatacttctaagatgtcaatgggaacacatctattggtgtgcatcaaggaattacatctattcactcacttatgatctgtaacccacaataaaacacccttttctccaaaaattaaccatatactataggcttctcagttgtatgagtgtgtgcgtatacacacatatacatacaccaaggtaatataccatatccacatataccaaggtaaaagattctttgtgtgggataaggaaacagcccagcgcttttacattaataatatcttgttcttaatttacagcgtttgtagcccttacctgagtgttatcattaaatatccagagattgaacttttcatcggggtaatgatataaaattgttccacaaagtgtactatatgaaccacttttcacagttcaaataacatattttagaaataaatatcataactagcaataacctatctacacaaggtggagaggatgagattaacaaaaaccaaattatatttccatatatctcatgttcaattcctaaatagcttgttttatttttcaaaatccaattgcacataacccataattgataggccacttcctctccaaaacaaataaactgtcaaagaataaagtgataaattataaaaaaggaaaatatgtatcatttactacagtcattccctttccccaaaacttggcaaacatataggaaaagtgctatcaagtgggtacactttgattataaatccaaagctcatttggagcagatgagattaataaaaataggacagaatgagtatatatttttatatacgtgagatgagtgcttgatttttacttaagaaatcaggaggatccatattaaatgggaaacaatggcatttatcaacaggagaacccattcatccagttactaccaaatctacaaattccaaatgtttctatcattcttatcatataaaagattggggcaaataaaattattgttattggttgtgtaaacttcaagctctctaagcttaaggctaatggtccttagggacatagttttatttggtgatcttcgcggggtgtacattagggccaaggttgcctttaaccaggttggtgtagtttttagggtgagggtaaggctcccagggtatgtgaaattcttctttaatagaggacaagggataaaatgcaaatccttctagttgaaacaaccaaatgacttaaatttatgctataaattaaatgattcatatcaattacttcattgagagcatgattttatggtagaaaataaactggggcctgaggcatggaggaagaggaatgtccgctaacacaaaggttatcaaatttagggtccctgggtggaatccctattccttttcggtcagatcttgttttaagctttattacgttgtcatgggatatctttcaaaatcctttactcaatcacatatggggggaaaattgcgttgaaatacagaattaaatcttaagtctttatggagatcgacaatttccatttttaaataaataaaatctatatgaatatcttcaacttcctaaagaaaaaagagagagaggaaaataaacttttgaacatgaaatcacttacataaacctcaagtgtactaacgtgtagaggaaaaaatctcaaatgtgggtgtaaccgctatacatttaggaaacatgccgccttgggagagtgcctataacgaattccgtctgccacccagtggccgctgaaataaattgtttcttttgttggccattgccctgtattttgctaaaaaaaaaaaaaaaaaaaagaggtagattatgccataccaggaatttaaagccatcaggacatgtgcctcgacatattttacaatacaatcagtgtagtaaatgttaaatattttccttttcgcgaactcagaggttaaccacgtggctctacgaataaataacgtgttcttcctgcgtccctgcatctacctgggctcagatactgactggcacagaagataccgaactggcccgggattcccgagtcacgttgttgggcatcgagagggtgcagcaggacacgccgacagtggcctcgggtagctcgtcgtcctccgtccactcgttgagctcggggctgaagcactggatgcacttcttgtacttcttctcgccctcgttccagccccccaccaggtaggcgcggccatgcagcgccgagacgcccgcagtgctcactcccacctgcagcggcgccgcgtagctccactggccggtcgcggggctgtagcactccacggtgagcacgtccacgcgctccccgcgcggccccagctggctgccgcccatcacgtacactctgtcgctcagcgtgaccgcgcagtgccagccccggggtgtgctgaggttcggcagctcctgccacgagtcgctggccgggtcgtaggcgcacacagagcgcgagtaggcgttggctatgtagcctccggtcaccagcacgcggccgtcggcgaccgcgctagcgtggcagcagcgcgccacctccaggggcgtcttcggctgccactgattggtggagggcacgtagcactccagcgaggccaggcttccttctgcgttgcggccgcccgcggcgtacacgagcccgttgaacacgctcaggctgaagtgcgtgcgcttctggttcatgctggccaggtgtatccaggtgttgaagcggggatcgtatctgcagaaattgctgactgcatgcttggcttgatttcttgcatcattctggtcttcaccaccggctacataaagaaatccatccatcacagccacacactgattaaaacttttggctggcatttccgtaagcttgctccatccattttcagggtctctatacaagatgtctctgctaagggacttctcagtaaggcctgggcgtcccccaacagtgacgaggactcggcagccacctcggattcttgttcgcctagattgcaatgtgttttgatgatatggaagcaagtggtagttcatagcatctacgagaagtctgtgacaatcagcatcttgcatcattcttggtacggattgaacataattgaccaggtcttgtgcagagatggtaccaaagcgaatattgctcaaaagatctgcagcgtattttactctcttttggtcaaattctaaccatttcattgcaatctggaatgctactatctcagaaggcaactgtaagtcatcatctataagaagttcattaatttgttcaaatgtaagtttcataaactgatccgattctgcaaattcaaggaagttatcccgaataaatttctgggctgctgcttttgcattttttagggagtatgtttcagcaatattaacaacatacatgcaattctcaacactcatctcccgtatcagaaaatcactgcacatctttacaagagtatggatctgaagataaacagcagcagaaataatgcttcctattgtatacaaggagagagtgagctttccagtgtaggcatatgcaatgacagtggccaggcctagtggtgagatatcattgagatccaccctctgaattgacgggtctttttttaggatgttgtaaaaatactcactgcatgaagccatgactgacttatgaacatcaaaggatttggttttggtaccaatgactaagtcacataggaagttctcctgccgcattttacttaaaccttccaagaggttggggccataagaagcatctgttagttcagaagaaatgcagctaaggccattgcctccctctaggagcccattcaaagcattcagtttgtttagggggctatcttctacgattatagtcatctcattgatatctcctttgttctttttgacaatcttctttttgggtgccatgttggcaaatacactgttacaggcaagagcttgcctccttgggtgaagtggcaggtcaacttgagatgatgaagttttagcaggagactcctcttgggaagggatctgtggagatagagagagggagaaggaaaatccggtggggagccaccagcagccacctgacaagacccggctgcagcaattttt

SEQ ID NO: 16628 - RNA, 1632 nt, Homo sapiens
  source 1..1632: mol_type = other RNA
gtgttctctgatggacagtaagagttcggttcaggctaaaggattttgcacattcattacattcatagggcttttctcctgtatgaattctctgatgctgaatgagaaataattgtgtactgaaggctttgccacactccttacagtcataaggtttctctccagaatgaattctctgatgctgaataaggtttgattgtctgttgaaggctttcccacattctttgcacttgtaaggtttctctccactatgaattctctgatgatgaattagattagagctatgactaaaggctttcccacactgattacactcatgatgtttctctcctgtatgaatttttagatgttgaacataagatgaatgtgtactaaaagctttcccacatttaatacactcatagggtttttctctagtgtgaattttacaatgctgaataaagtatgagtgaacactgaaagatttgccacaatcctcacatgtgtagagtttcttaccagtgtggattctctgatgtttactgaggatagagggccaactgaaagcttttccacattcattgtgctcataggtcttctctccactatgaaatctctggtgctggttaaaagctctgttctgattgtaagtttttccacacccagtactctcaaaccatctctctggattattcatcctctgattctcactaagaactgagctctgtctgggcactttcactaacacatctgtctgataggctctttctcctaattggaaactctggaggttaatgaggtcctcatgttgttgcaagttttctacacttgacacacttggatggagactctcctctctagaccctctaagatgtttggcaggatttgagtctgtaatgcagttttctccaacagcattgaacttctggccattctctctagagagggttttcacatacctcatggtaatttctctgaaattgctcttctgggagaatgagttcttaactccttctactgcatattttctccagcaattctctaactttccctcagttttactcatctcttcagtttccttaaaaatattccttacatgatcttctgattttgctctctgggattccaattcttcagaaatgtcctgctttggaatcatttcctctttttcaatcctagaatcacagccttctctcttgtgcctccagctccagctcccctgagttctcaggatgtgaggggtctatggttcgtccccccgctccagcctggagatgacatcaggtttggaagcttgaagtcatgcatatattgcatcgtggtgaagtctgggcagttccttttgattgttgagtcgtatcccatggtatggatgtaccacagtttgcttaaccattcacctactaatgagagtaggttcccataggtccccatcatcacatccttgtagaggcccctctgagcagggatcagacagtcccactcctcctgggagaggggtacagccacatcctcaaaggaaaccacgatgtggaatgacaagatcttgatgcagccctcaggtcaggactcggctcgaccacgggaagggaaggagcgcgaacgctaaatcccgtgccgcggggagccaagccccctgggccggaaatgcct

SEQ ID NO: 16629 - RNA, 1482 nt, Homo sapiens
  source 1..1482: mol_type = other RNA
gtgttctctgatggacagtaagccttgacttatggctaaatgcttcttcacaatggtcacatgcatagggcttttcccctgtgtgagttctatgatgtattgtgaggtatgacttctggctaaaggtttttccacattcactacactgatagggcttttcccctgagtgagttctgtgatgtaaagtgagaagtgacttacagtgaaaagtttttccacattcaatacatttgtagggtttatcccctgtgtgagttctctcatgtaaagtgaggaatgacttacggcgaaaggttttaccacattcattgcatccatagggcttttcccctgtgtgaattctctgatggataatgaggctggacttatagctgaacaatttttcacaccagttacaggcataaggtttttcctcagtaggcatcttgcactgtagcataaggtctgatttgctaatggagggtttctcacattcaacacattcatagggtttctctcctgtgtgtgtctgctgatgtttagtgaagtcagactttctacagcaagttggctgtcctacctgagttatcacttggacaataacagctgagttattacaggctttctcatattcattatatttaccaaaggtctgtactatatgaaccctcttatgtataaagaacattgcctccgtgttgaaggttttcccttgttcattacattgaaaagtctgcagcagagtttgaatcttgtgatgctgagtaagatgttcatgatgtctgtgggatctcctggttatatcacagacatgaggtttctctccagactgtgtctccccaggcttaatagggaaaagcatgttctggcaatcattaaactgcccaggcttcattcctgaactgtttccattatttataatcagatttaaaacatggtttgagttcaaattaaatgtttttcctaattcaactctctcctgagttgatgtgttgctgttggtgattacaatttgccagaaaaatctatcatgactttcatggctcctttcaataaggtcatcaatgatctggacagctgaaagtctcaggtttggggtttcttctactatccatggctctgctccttgctctagcttgaagatcatctcaggtttggtaatgtaatgccccaatgataccaggctgctgtaggtctccagcatcacgtccctgtacagggtcctctgagcatcatccaggtcctgccactcctcccaggtgaagtgcacagctacctcctcaaaggacaccaactccagagatttattcttttcttgtagctcttggaaacagccagagaacactggaaacatagccttaaggctgaagaccatcatccagtaccccatctccctcgcggcatcagtgagttcttccctggaaactaggtctcgtataaacttccgcagggacatagaaccaagccccaggctggcccagctacaagaccgcctctgggtgc

SEQ ID NO: 16630 - RNA, 1483 nt, Homo sapiens
  source 1..1483: mol_type = other RNA
gtgttctctgatggacagtaagccttgacttatggctaaatgcttcttcacaatggtcacatgcatagggcttttcccctgtgtgagttctatgatgtattgtgaggtatgacttctggctaaaggtttttccacattcactacactgatagggcttttcccctgagtgagttctgtgatgtaaagtgagaagtgacttacagtgaaaagtttttccacattcaatacatttgtagggtttatcccctgtgtgagttctctcatgtaaagtgaggaatgacttacggcgaaaggttttaccacattcattgcatccatagggcttttcccctgtgtgaattctctgatggataatgaggctggacttatagctgaacaatttttcacaccagttacaggcataaggtttttcctcagtaggcatcttgcactgtagcataaggtctgatttgctaatggagggtttctcacattcaacacattcatagggtttctctcctgtgtgtgtctgctgatgtttagtgaagtcagactttctacagcaagttggctgtcctacctgagttatcacttggacaataacagctgagttattacaggctttctcatattcattatatttaccaaaggtctgtactatatgaaccctcttatgtataaagaacattgcctccgtgttgaaggttttcccttgttcattacattgaaaagtctgcagcagagtttgaatcttgtgatgctgagtaagatgttcatgatgtctgtgggatctcctggttatatcacagacatgaggtttctctccagactgtgtctccccaggcttaatagggaaaagcatgttctggcaatcattaaactgcccaggcttcattcctgaactgtttccattatttataatcagatttaaaacatggtttgagttcaaattaaatgtttttcctaattcaactctctcctgagttgatgtgttgctgttggtgattacaatttgccagaaaaatctatcatgactttcatggctcctttcaataaggtcatcaatgatctggacagctgaaagtctcaggtttggggtttcttctactatccatggctctgctccttgctctagcttgaagatcatctcaggtttggtaatgtaatgccccaatgataccaggctgctgtaggtctccagcatcacgtccctgtacagggtcctctgagcatcatccaggtcctgccactcctcccaggtgaagtgcacagctacctcctcaaaggacaccaactccagagatttattcttttcttgtagctcttggaaacagccagagaacactggaaacatagccttaaggctgaagaccatcatccagtaccccatctccctcgcggcatcagtgagttcttccctggaaactaggtctcgtataaacttccgcagggacatagaaccaagccccaggctggcccagctacaagaccgcctctgggtgcc

SEQ ID NO: 16631 - RNA, 1484 nt, Homo sapiens
  source 1..1484: mol_type = other RNA
gtgttctctgatggacagtaagccttgacttatggctaaatgcttcttcacaatggtcacatgcatagggcttttcccctgtgtgagttctatgatgtattgtgaggtatgacttctggctaaaggtttttccacattcactacactgatagggcttttcccctgagtgagttctgtgatgtaaagtgagaagtgacttacagtgaaaagtttttccacattcaatacatttgtagggtttatcccctgtgtgagttctctcatgtaaagtgaggaatgacttacggcgaaaggttttaccacattcattgcatccatagggcttttcccctgtgtgaattctctgatggataatgaggctggacttatagctgaacaatttttcacaccagttacaggcataaggtttttcctcagtaggcatcttgcactgtagcataaggtctgatttgctaatggagggtttctcacattcaacacattcatagggtttctctcctgtgtgtgtctgctgatgtttagtgaagtcagactttctacagcaagttggctgtcctacctgagttatcacttggacaataacagctgagttattacaggctttctcatattcattatatttaccaaaggtctgtactatatgaaccctcttatgtataaagaacattgcctccgtgttgaaggttttcccttgttcattacattgaaaagtctgcagcagagtttgaatcttgtgatgctgagtaagatgttcatgatgtctgtgggatctcctggttatatcacagacatgaggtttctctccagactgtgtctccccaggcttaatagggaaaagcatgttctggcaatcattaaactgcccaggcttcattcctgaactgtttccattatttataatcagatttaaaacatggtttgagttcaaattaaatgtttttcctaattcaactctctcctgagttgatgtgttgctgttggtgattacaatttgccagaaaaatctatcatgactttcatggctcctttcaataaggtcatcaatgatctggacagctgaaagtctcaggtttggggtttcttctactatccatggctctgctccttgctctagcttgaagatcatctcaggtttggtaatgtaatgccccaatgataccaggctgctgtaggtctccagcatcacgtccctgtacagggtcctctgagcatcatccaggtcctgccactcctcccaggtgaagtgcacagctacctcctcaaaggacaccaactccagagatttattcttttcttgtagctcttggaaacagccagagaacactggaaacatagccttaaggctgaagaccatcatccagtaccccatctccctcgcggcatcagtgagttcttccctggaaactaggtctcgtataaacttccgcagggacatagaaccaagccccaggctggcccagctacaagaccgcctctgggtgccg

SEQ ID NO: 16632 - RNA, 1618 nt, Homo sapiens
  source 1..1618: mol_type = other RNA
gtgttctctgatggacagtaagccttgacttatggctaaatgcttcttcacaatggtcacatgcatagggcttttcccctgtgtgagttctatgatgtattgtgaggtatgacttctggctaaaggtttttccacattcactacactgatagggcttttcccctgagtgagttctgtgatgtaaagtgagaagtgacttacagtgaaaagtttttccacattcaatacatttgtagggtttatcccctgtgtgagttctctcatgtaaagtgaggaatgacttacggcgaaaggttttaccacattcattgcatccatagggcttttcccctgtgtgaattctctgatggataatgaggctggacttatagctgaacaatttttcacaccagttacaggcataaggtttttcctcagtaggcatcttgcactgtagcataaggtctgatttgctaatggagggtttctcacattcaacacattcatagggtttctctcctgtgtgtgtctgctgatgtttagtgaagtcagactttctacagcaagttggctgtcctacctgagttatcacttggacaataacagctgagttattacaggctttctcatattcattatatttaccaaaggtctgtactatatgaaccctcttatgtataaagaacattgcctccgtgttgaaggttttcccttgttcattacattgaaaagtctgcagcagagtttgaatcttgtgatgctgagtaagatgttcatgatgtctgtgggatctcctggttatatcacagacatgaggtttctctccagactgtgtctccccaggcttaatagggaaaagcatgttctggcaatcattaaactgcccaggcttcattcctgaactgtttccattatttataatcagatttaaaacatggtttgagttcaaattaaatgtttttcctaattcaactctctcctgagttgatgtgttgctgttggtgattacaatttgccagaaaaatctatcatgactttcatggctcctttcaataaggtcatcaatgatctggacagctgaaagtctcaggtttggggtttcttctactatccatggctctgctccttgctctagcttgaagatcatctcaggtttggtaatgtaatgccccaatgataccaggctgctgtaggtctccagcatcacgtccctgtacagggtcctctgagcatcatccaggtcctgccactcctcccaggtgaagtgcacagctacctcctcaaaggacaccaactccagagatttattcttttcttgtagctcttggaaacagccagagaacactggaaacatagccttaaggctgaagaccatcatccagtaccccatctccctcgcggcatcagtgagttcttccctggaaactaggtctcgtataaacttctgcacttcaggccctgcccgcccgcgatgcgcccacgcgtctgctcccacaactggggaacactggtccggccccccgggatcccccgggcccacgggttcctcttcgccctcgcaccgacccgcagggacatagaaccaagccccaggctggcccagctacaagaccgcctctgggtgccgcacttccggagg

SEQ ID NO: 16633 - RNA, 1501 nt, Homo sapiens
  source 1..1501: mol_type = other RNA
gtgttctctgatggacagtaagccttgacttatggctaaatgcttcttcacaatggtcacatgcatagggcttttcccctgtgtgagttctatgatgtattgtgaggtatgacttctggctaaaggtttttccacattcactacactgatagggcttttcccctgagtgagttctgtgatgtaaagtgagaagtgacttacagtgaaaagtttttccacattcaatacatttgtagggtttatcccctgtgtgagttctctcatgtaaagtgaggaatgacttacggcgaaaggttttaccacattcattgcatccatagggcttttcccctgtgtgaattctctgatggataatgaggctggacttatagctgaacaatttttcacaccagttacaggcataaggtttttcctcagtaggcatcttgcactgtagcataaggtctgatttgctaatggagggtttctcacattcaacacattcatagggtttctctcctgtgtgtgtctgctgatgtttagtgaagtcagactttctacagcaagttggctgtcctacctgagttatcacttggacaataacagctgagttattacaggctttctcatattcattatatttaccaaaggtctgtactatatgaaccctcttatgtataaagaacattgcctccgtgttgaaggttttcccttgttcattacattgaaaagtctgcagcagagtttgaatcttgtgatgctgagtaagatgttcatgatgtctgtgggatctcctggttatatcacagacatgaggtttctctccagactgtgtctccccaggcttaatagggaaaagcatgttctggcaatcattaaactgcccaggcttcattcctgaactgtttccattatttataatcagatttaaaacatggtttgagttcaaattaaatgtttttcctaattcaactctctcctgagttgatgtgttgctgttggtgattacaatttgccagaaaaatctatcatgactttcatggctcctttcaataaggtcatcaatgatctggacagctgaaagtctcaggtttggggtttcttctactatccatggctctgctccttgctctagcttgaagatcatctcaggtttggtaatgtaatgccccaatgataccaggctgctgtaggtctccagcatcacgtccctgtacagggtcctctgagcatcatccaggtcctgccactcctcccaggtgaagtgcacagctacctcctcaaaggacaccaactccagagatttattcttttcttgtagctcttggaaacagccagagaacactggaaacatagctgcacttcaggccctgcccgcccgcgatgcgcccacgcgtctgctcccacaactggggaacactggtccggccccccgggatcccccgggcccacgggttcctcttcgccctcgcaccgacccgcagggacatagaaccaagccccaggctggcccagctacaag

SEQ ID NO: 16634 - RNA, 1632 nt, Homo sapiens
  source 1..1632: mol_type = other RNA
gtgttctctgatggacagtaagccttgacttatggctaaatgcttcttcacaatggtcacatgcatagggcttttcccctgtgtgagttctatgatgtattgtgaggtatgacttctggctaaaggtttttccacattcactacactgatagggcttttcccctgagtgagttctgtgatgtaaagtgagaagtgacttacagtgaaaagtttttccacattcaatacatttgtagggtttatcccctgtgtgagttctctcatgtaaagtgaggaatgacttacggcgaaaggttttaccacattcattgcatccatagggcttttcccctgtgtgaattctctgatggataatgaggctggacttatagctgaacaatttttcacaccagttacaggcataaggtttttcctcagtaggcatcttgcactgtagcataaggtctgatttgctaatggagggtttctcacattcaacacattcatagggtttctctcctgtgtgtgtctgctgatgtttagtgaagtcagactttctacagcaagttggctgtcctacctgagttatcacttggacaataacagctgagttattacaggctttctcatattcattatatttaccaaaggtctgtactatatgaaccctcttatgtataaagaacattgcctccgtgttgaaggttttcccttgttcattacattgaaaagtctgcagcagagtttgaatcttgtgatgctgagtaagatgttcatgatgtctgtgggatctcctggttatatcacagacatgaggtttctctccagactgtgtctccccaggcttaatagggaaaagcatgttctggcaatcattaaactgcccaggcttcattcctgaactgtttccattatttataatcagatttaaaacatggtttgagttcaaattaaatgtttttcctaattcaactctctcctgagttgatgtgttgctgttggtgattacaatttgccagaaaaatctatcatgactttcatggctcctttcaataaggtcatcaatgatctggacagctgaaagtctcaggtttggggtttcttctactatccatggctctgctccttgctctagcttgaagatcatctcaggtttggtaatgtaatgccccaatgataccaggctgctgtaggtctccagcatcacgtccctgtacagggtcctctgagcatcatccaggtcctgccactcctcccaggtgaagtgcacagctacctcctcaaaggacaccaactccagagatttattcttttcttgtagctcttggaaacagccagagaacactggaaacatagctgtgaccttttatcctcctctgaagcaccagtgggaggttagaccagagggctgttctttcaagtgcgcttcttattcatagggaaccctccctttcaaacctgcacttcaggccctgcccgcccgcgatgcgcccacgcgtctgctcccacaactggggaacactggtccggccccccgggatcccccgggcccacgggttcctcttcgccctcgcaccgacccgcagggacatagaaccaagccccaggctggcccagctacaagaccgcctctgggtgccgcacttccggagg

SEQ ID NO: 16635 - RNA, 1554 nt, Homo sapiens
  source 1..1554: mol_type = other RNA
gtgttctctgatggacagtaagccttgacttatggctaaatgcttcttcacaatggtcacatgcatagggcttttcccctgtgtgagttctatgatgtattgtgaggtatgacttctggctaaaggtttttccacattcactacactgatagggcttttcccctgagtgagttctgtgatgtaaagtgagaagtgacttacagtgaaaagtttttccacattcaatacatttgtagggtttatcccctgtgtgagttctctcatgtaaagtgaggaatgacttacggcgaaaggttttaccacattcattgcatccatagggcttttcccctgtgtgaattctctgatggataatgaggctggacttatagctgaacaatttttcacaccagttacaggcataaggtttttcctcagtaggcatcttgcactgtagcataaggtctgatttgctaatggagggtttctcacattcaacacattcatagggtttctctcctgtgtgtgtctgctgatgtttagtgaagtcagactttctacagcaagttggctgtcctacctgagttatcacttggacaataacagctgagttattacaggctttctcatattcattatatttaccaaaggtctgtactatatgaaccctcttatgtataaagaacattgcctccgtgttgaaggttttcccttgttcattacattgaaaagtctgcagcagagtttgaatcttgtgatgctgagtaagatgttcatgatgtctgtgggatctcctggttatatcacagacatgaggtttctctccagactgtgtctccccaggcttaatagggaaaagcatgttctggcaatcattaaactgcccaggcttcattcctgaactgtttccattatttataatcagatttaaaacatggtttgagttcaaattaaatgtttttcctaattcaactctctcctgagttgatgtgttgctgttggtgattacaatttgccagaaaaatctatcatgactttcatggctcctttcaataaggtcatcaatgatctggacagctgaaagtctcaggtttggggtttcttctactatccatggctctgctccttgctctagcttgaagatcatctcaggtttggtaatgtaatgccccaatgataccaggctgctgtaggtctccagcatcacgtccctgtacagggtcctctgagcatcatccaggtcctgccactcctcccaggtgaagtgcacagctacctcctcaaaggacaccaactccagagatttattcttttcttgtagctcttggaaacagccagagaacactggaaacatagctgtgaccttttatcctcctctgaagcaccagtgggaggttagaccagagggctgttctttcaagtgcgcttcttattcatagggaaccctccctttcaaaccttataacacacggttaagactgaagtacccttaaggctgaagaccatcatccagtaccccatctccctcgcggcatcagtgagttcttccctggaaactaggtctcgtataaactt

SEQ ID NO: 16636 - RNA, 1530 nt, Homo sapiens
  source 1..1530: mol_type = other RNA
gtgttctctgatggacagtaagccttgacttatggctaaatgcttcttcacaatggtcacatgcatagggcttttcccctgtgtgagttctatgatgtattgtgaggtatgacttctggctaaaggtttttccacattcactacactgatagggcttttcccctgagtgagttctgtgatgtaaagtgagaagtgacttacagtgaaaagtttttccacattcaatacatttgtagggtttatcccctgtgtgagttctctcatgtaaagtgaggaatgacttacggcgaaaggttttaccacattcattgcatccatagggcttttcccctgtgtgaattctctgatggataatgaggctggacttatagctgaacaatttttcacaccagttacaggcataaggtttttcctcagtaggcatcttgcactgtagcataaggtctgatttgctaatggagggtttctcacattcaacacattcatagggtttctctcctgtgtgtgtctgctgatgtttagtgaagtcagactttctacagcaagttggctgtcctacctgagttatcacttggacaataacagctgagttattacaggctttctcatattcattatatttaccaaaggtctgtactatatgaaccctcttatgtataaagaacattgcctccgtgttgaaggttttcccttgttcattacattgaaaagtctgcagcagagtttgaatcttgtgatgctgagtaagatgttcatgatgtctgtgggatctcctggttatatcacagacatgaggtttctctccagactgtgtctccccaggcttaatagggaaaagcatgttctggcaatcattaaactgcccaggcttcattcctgaactgtttccattatttataatcagatttaaaacatggtttgagttcaaattaaatgtttttcctaattcaactctctcctgagttgatgtgttgctgttggtgattacaatttgccagaaaaatctatcatgactttcatggctcctttcaataaggtcatcaatgatctggacagctgaaagtctcaggtttggggtttcttctactatccatggctctgctccttgctctagcttgaagatcatctcaggtttggtaatgtaatgccccaatgataccaggctgctgtaggtctccagcatcacgtccctgtacagggtcctctgagcatcatccaggtcctgccactcctcccaggtgaagtgcacagctacctcctcaaaggacaccaactcccttaaggctgaagaccatcatccagtaccccatctccctcgcggcatcagtgagttcttccctggaaactaggtctcgtataaacttctgcacttcaggccctgcccgcccgcgatgcgcccacgcgtctgctcccacaactggggaacactggtccggccccccgggatcccccgggcccacgggttcctcttcgccctcgcaccgacccgcagggacatagaaccaagccccaggctggcccagctacaag

SEQ ID NO: 16637 - RNA, 1600 nt, Homo sapiens
  source 1..1600: mol_type = other RNA
gtgttctctgatggacagtaagccttgacttatggctaaatgcttcttcacaatggtcacatgcatagggcttttcccctgtgtgagttctatgatgtattgtgaggtatgacttctggctaaaggtttttccacattcactacactgatagggcttttcccctgagtgagttctgtgatgtaaagtgagaagtgacttacagtgaaaagtttttccacattcaatacatttgtagggtttatcccctgtgtgagttctctcatgtaaagtgaggaatgacttacggcgaaaggttttaccacattcattgcatccatagggcttttcccctgtgtgaattctctgatggataatgaggctggacttatagctgaacaatttttcacaccagttacaggcataaggtttttcctcagtaggcatcttgcactgtagcataaggtctgatttgctaatggagggtttctcacattcaacacattcatagggtttctctcctgtgtgtgtctgctgatgtttagtgaagtcagactttctacagcaagttggctgtcctacctgagttatcacttggacaataacagctgagttattacaggctttctcatattcattatatttaccaaaggtctgtactatatgaaccctcttatgtataaagaacattgcctccgtgttgaaggttttcccttgttcattacattgaaaagtctgcagcagagtttgaatcttgtgatgctgagtaagatgttcatgatgtctgtgggatctcctggttatatcacagacatgaggtttctctccagactgtgtctccccaggcttaatagggaaaagcatgttctggcaatcattaaactgcccaggcttcattcctgaactgtttccattatttataatcagatttaaaacatggtttgagttcaaattaaatgtttttcctaattcaactctctcctgagttgatgtgttgctgttggtgattacaatttgccagaaaaatctatcatgactttcatggctcctttcaataaggtcatcaatgatctggacagctgaaagtctcaggtttggggtttcttctactatccatggctctgctccttgctctagcttgaagatcatctcaggtttggtaatgtaatgccccaatgataccaggctgctgtaggtctccagcatcacgtccctgtacagggtcctctgagcatcatccaggtcctgccactcctcccaggtgaagtgcacagctacctcctcaaaggacaccaactcctgtaatgataccaggctgttgtaggtctccagcatcacgttcctgtacagggtcctctaagcatcatccacgtcctgccactcctcccaggtgaagtgcacagccacatcttcaaaggacaccaaccccagagatttattcttttcttgtagctcttggaaacagccagagaacactggaaacatagctgcacttcaggccctgcccgcccgcgatgcgcccacgcgtctgctcccacaactggggaacactggtccggccccccgggatcccccgggcccacgggttcctcttcgccctcgcaccgacccgcagggacatag

SEQ ID NO: 16638 - RNA, 2259 nt, Homo sapiens
  source 1..2259: mol_type = other RNA
gtgttctctgatggacagtaagccttgacttatggctaaatgcttcttcacaatggtcacatgcatagggcttttcccctgtgtgagttctatgatgtattgtgaggtatgacttctggctaaaggtttttccacattcactacactgatagggcttttcccctgagtgagttctgtgatgtaaagtgagaagtgacttacagtgaaaagtttttccacattcaatacatttgtagggtttatcccctgtgtgagttctctcatgtaaagtgaggaatgacttacggcgaaaggttttaccacattcattgcatccatagggcttttcccctgtgtgaattctctgatggataatgaggctggacttatagctgaacaatttttcacaccagttacaggcataaggtttttcctcagtaggcatcttgcactgtagcataaggtctgatttgctaatggagggtttctcacattcaacacattcatagggtttctctcctgtgtgtgtctgctgatgtttagtgaagtcagactttctacagcaagttggctgtcctacctgagttatcacttggacaataacagctgagttattacaggctttctcatattcattatatttaccaaaggtctgtactatatgaaccctcttatgtataaagaacattgcctccgtgttgaaggttttcccttgttcattacattgaaaagtctgcagcagagtttgaatcttgtgatgctgagtaagatgttcatgatgtctgtgggatctcctggttatatcacagacatgaggtttctctccagactgtgtctccccaggcttaatagggaaaagcatgttctggcaatcattaaactgcccaggcttcattcctgaactgtttccattatttataatcagatttaaaacatggtttgagttcaaattaaatgtttttcctaattcaactctctcctgagttgatgtgttgctgttggtgattacaatttgccagaaaaatctatcatgactttcatggctcctttcaataaggtcatcaatgatctggacagctgaaagtctcaggtttggggtttcttctactatccatggctctgctccttgctctagcttgaagatcatctcaggtttggtaatgtaatgccccaatgataccaggctgctgtaggtctccagcatcacgtccctgtacagggtcctctgagcatcatccaggtcctgccactcctcccaggtgaagtgcacagctacctcctcaaaggacaccaactcctgtaatgataccaggctgttgtaggtctccagcatcacgttcctgtacagggtcctctaagcatcatccacgtcctgccactcctcccaggtgaagtgcacagccacatcttcaaaggacaccaaccccagagatttattcttttcttgtagctcttggaaacagccagagaacactggaaacatagctgtgaccttttatcctcctctgaagcaccagtgggaggttagaccagagggctgttctttcaagtgcgcttcttattcatagggaaccctccctttcaaaccttataacacacggttaagactgaagtacccttaaggctgaagaccatcatccagtaccccatctccctcgcggcatcagtgagttcttccctggaaactaggtctcgtataaacttctgtaaacgcaacccaggaggactaggcaggtcacacagtgaaggagggaaccagaaacttcacttgctaaagagacaccgggaaacccaactaatacaaacgcccagtttaagactcgaggcgcacgcgtttcgcactactcctctgggaatggggaacgtctcccgagaactgtgtgttcgcactgggacagatgggcaaactgagcgtcatgcgggttggtaaccggctccctcagcggcaggacaggagcgcggcctgcagactccgggcccagggccaccggcctcgcctacccgctcctgcgcctctagaacccgcttcactgccgggaccccacgcctgtcctcccagcccccgccagggtccgcggcctgcacctgcacttcaggccctgcccgcccgcgatgcgcccacgcgtctgctcccacaactggggaacactggtccggccccccgggatcccccgggcccacgggttcctcttcgccctcgcaccgacccgcagggacatagaaccaagccccaggctggcccagctacaagaccgcctctgggtgccgcacttccggagg

SEQ ID NO: 16639 - RNA, 1734 nt, Homo sapiens
  source 1..1734: mol_type = other RNA
gtgttctctgatggacagtgaggaatgacttacagcgaaaggttttcccacattcattgcattcgtagggtttttcccctgtgtgagtccattgatggatagtgaggaatgacttacggtgaaacgttttcccacattcattgcattcatagggtttttcccctgtgtgagttctctgatgtaacctgaggtttgacttattgataaagggttttccacactcattacattcatacggtttttcccctgtgtgtgttctctgatggacagtaagccttgacttatggctaaatgcttcttcacaatggtcacatgcatagggcttttcccctgtgtgagttctatgatgtattgtgaggtatgacttctggctaaaggtttttccacattcactacactgatagggcttttcccctgagtgagttctgtgatgtaaagtgagaagtgacttacagtgaaaagtttttccacattcaatacatttgtagggtttatcccctgtgtgagttctctcatgtaaagtgaggaatgacttacggcgaaaggttttaccacattcattgcatccatagggcttttcccctgtgtgaattctctgatggataatgaggctggacttatagctgaacaatttttcacaccagttacaggcataaggtttttcctcagtaggcatcttgcactgtagcataaggtctgatttgctaatggagggtttctcacattcaacacattcatagggtttctctcctgtgtgtgtctgctgatgtttagtgaagtcagactttctacagcaagttggctgtcctacctgagttatcacttggacaataacagctgagttattacaggctttctcatattcattatatttaccaaaggtctgtactatatgaaccctcttatgtataaagaacattgcctccgtgttgaaggttttcccttgttcattacattgaaaagtctgcagcagagtttgaatcttgtgatgctgagtaagatgttcatgatgtctgtgggatctcctggttatatcacagacatgaggtttctctccagactgtgtctccccaggcttaatagggaaaagcatgttctggcaatcattaaactgcccaggcttcattcctgaactgtttccattatttataatcagatttaaaacatggtttgagttcaaattaaatgtttttcctaattcaactctctcctgagttgatgtgttgctgttggtgattacaatttgccagaaaaatctatcatgactttcatggctcctttcaataaggtcatcaatgatctggacagctgaaagtctcaggtttggggtttcttctactatccatggctctgctccttgctctagcttgaagatcatctcaggtttggtaatgtaatgccccaatgataccaggctgctgtaggtctccagcatcacgtccctgtacagggtcctctgagcatcatccaggtcctgccactcctcccaggtgaagtgcacagctacctcctcaaaggacaccaactccagagatttattcttttcttgtagctcttggaaacagccagagaacactggaaacatagccttaaggctgaagaccatcatccagtaccccatctccctcgcggcatcagtgagttcttccctggaaactaggtctcgtataaacttccgcagggacatagaaccaagccccaggctggcccagctacaagaccgcctctgggtgc

SEQ ID NO: 16640 - RNA, 1735 nt, Homo sapiens
  source 1..1735: mol_type = other RNA
gtgttctctgatggacagtgaggaatgacttacagcgaaaggttttcccacattcattgcattcgtagggtttttcccctgtgtgagtccattgatggatagtgaggaatgacttacggtgaaacgttttcccacattcattgcattcatagggtttttcccctgtgtgagttctctgatgtaacctgaggtttgacttattgataaagggttttccacactcattacattcatacggtttttcccctgtgtgtgttctctgatggacagtaagccttgacttatggctaaatgcttcttcacaatggtcacatgcatagggcttttcccctgtgtgagttctatgatgtattgtgaggtatgacttctggctaaaggtttttccacattcactacactgatagggcttttcccctgagtgagttctgtgatgtaaagtgagaagtgacttacagtgaaaagtttttccacattcaatacatttgtagggtttatcccctgtgtgagttctctcatgtaaagtgaggaatgacttacggcgaaaggttttaccacattcattgcatccatagggcttttcccctgtgtgaattctctgatggataatgaggctggacttatagctgaacaatttttcacaccagttacaggcataaggtttttcctcagtaggcatcttgcactgtagcataaggtctgatttgctaatggagggtttctcacattcaacacattcatagggtttctctcctgtgtgtgtctgctgatgtttagtgaagtcagactttctacagcaagttggctgtcctacctgagttatcacttggacaataacagctgagttattacaggctttctcatattcattatatttaccaaaggtctgtactatatgaaccctcttatgtataaagaacattgcctccgtgttgaaggttttcccttgttcattacattgaaaagtctgcagcagagtttgaatcttgtgatgctgagtaagatgttcatgatgtctgtgggatctcctggttatatcacagacatgaggtttctctccagactgtgtctccccaggcttaatagggaaaagcatgttctggcaatcattaaactgcccaggcttcattcctgaactgtttccattatttataatcagatttaaaacatggtttgagttcaaattaaatgtttttcctaattcaactctctcctgagttgatgtgttgctgttggtgattacaatttgccagaaaaatctatcatgactttcatggctcctttcaataaggtcatcaatgatctggacagctgaaagtctcaggtttggggtttcttctactatccatggctctgctccttgctctagcttgaagatcatctcaggtttggtaatgtaatgccccaatgataccaggctgctgtaggtctccagcatcacgtccctgtacagggtcctctgagcatcatccaggtcctgccactcctcccaggtgaagtgcacagctacctcctcaaaggacaccaactccagagatttattcttttcttgtagctcttggaaacagccagagaacactggaaacatagccttaaggctgaagaccatcatccagtaccccatctccctcgcggcatcagtgagttcttccctggaaactaggtctcgtataaacttccgcagggacatagaaccaagccccaggctggcccagctacaagaccgcctctgggtgcc

SEQ ID NO: 16641 - RNA, 1736 nt, Homo sapiens
  source 1..1736: mol_type = other RNA
gtgttctctgatggacagtgaggaatgacttacagcgaaaggttttcccacattcattgcattcgtagggtttttcccctgtgtgagtccattgatggatagtgaggaatgacttacggtgaaacgttttcccacattcattgcattcatagggtttttcccctgtgtgagttctctgatgtaacctgaggtttgacttattgataaagggttttccacactcattacattcatacggtttttcccctgtgtgtgttctctgatggacagtaagccttgacttatggctaaatgcttcttcacaatggtcacatgcatagggcttttcccctgtgtgagttctatgatgtattgtgaggtatgacttctggctaaaggtttttccacattcactacactgatagggcttttcccctgagtgagttctgtgatgtaaagtgagaagtgacttacagtgaaaagtttttccacattcaatacatttgtagggtttatcccctgtgtgagttctctcatgtaaagtgaggaatgacttacggcgaaaggttttaccacattcattgcatccatagggcttttcccctgtgtgaattctctgatggataatgaggctggacttatagctgaacaatttttcacaccagttacaggcataaggtttttcctcagtaggcatcttgcactgtagcataaggtctgatttgctaatggagggtttctcacattcaacacattcatagggtttctctcctgtgtgtgtctgctgatgtttagtgaagtcagactttctacagcaagttggctgtcctacctgagttatcacttggacaataacagctgagttattacaggctttctcatattcattatatttaccaaaggtctgtactatatgaaccctcttatgtataaagaacattgcctccgtgttgaaggttttcccttgttcattacattgaaaagtctgcagcagagtttgaatcttgtgatgctgagtaagatgttcatgatgtctgtgggatctcctggttatatcacagacatgaggtttctctccagactgtgtctccccaggcttaatagggaaaagcatgttctggcaatcattaaactgcccaggcttcattcctgaactgtttccattatttataatcagatttaaaacatggtttgagttcaaattaaatgtttttcctaattcaactctctcctgagttgatgtgttgctgttggtgattacaatttgccagaaaaatctatcatgactttcatggctcctttcaataaggtcatcaatgatctggacagctgaaagtctcaggtttggggtttcttctactatccatggctctgctccttgctctagcttgaagatcatctcaggtttggtaatgtaatgccccaatgataccaggctgctgtaggtctccagcatcacgtccctgtacagggtcctctgagcatcatccaggtcctgccactcctcccaggtgaagtgcacagctacctcctcaaaggacaccaactccagagatttattcttttcttgtagctcttggaaacagccagagaacactggaaacatagccttaaggctgaagaccatcatccagtaccccatctccctcgcggcatcagtgagttcttccctggaaactaggtctcgtataaacttccgcagggacatagaaccaagccccaggctggcccagctacaagaccgcctctgggtgccg

SEQ ID NO: 16642 - RNA, 1870 nt, Homo sapiens
  source 1..1870: mol_type = other RNA
gtgttctctgatggacagtgaggaatgacttacagcgaaaggttttcccacattcattgcattcgtagggtttttcccctgtgtgagtccattgatggatagtgaggaatgacttacggtgaaacgttttcccacattcattgcattcatagggtttttcccctgtgtgagttctctgatgtaacctgaggtttgacttattgataaagggttttccacactcattacattcatacggtttttcccctgtgtgtgttctctgatggacagtaagccttgacttatggctaaatgcttcttcacaatggtcacatgcatagggcttttcccctgtgtgagttctatgatgtattgtgaggtatgacttctggctaaaggtttttccacattcactacactgatagggcttttcccctgagtgagttctgtgatgtaaagtgagaagtgacttacagtgaaaagtttttccacattcaatacatttgtagggtttatcccctgtgtgagttctctcatgtaaagtgaggaatgacttacggcgaaaggttttaccacattcattgcatccatagggcttttcccctgtgtgaattctctgatggataatgaggctggacttatagctgaacaatttttcacaccagttacaggcataaggtttttcctcagtaggcatcttgcactgtagcataaggtctgatttgctaatggagggtttctcacattcaacacattcatagggtttctctcctgtgtgtgtctgctgatgtttagtgaagtcagactttctacagcaagttggctgtcctacctgagttatcacttggacaataacagctgagttattacaggctttctcatattcattatatttaccaaaggtctgtactatatgaaccctcttatgtataaagaacattgcctccgtgttgaaggttttcccttgttcattacattgaaaagtctgcagcagagtttgaatcttgtgatgctgagtaagatgttcatgatgtctgtgggatctcctggttatatcacagacatgaggtttctctccagactgtgtctccccaggcttaatagggaaaagcatgttctggcaatcattaaactgcccaggcttcattcctgaactgtttccattatttataatcagatttaaaacatggtttgagttcaaattaaatgtttttcctaattcaactctctcctgagttgatgtgttgctgttggtgattacaatttgccagaaaaatctatcatgactttcatggctcctttcaataaggtcatcaatgatctggacagctgaaagtctcaggtttggggtttcttctactatccatggctctgctccttgctctagcttgaagatcatctcaggtttggtaatgtaatgccccaatgataccaggctgctgtaggtctccagcatcacgtccctgtacagggtcctctgagcatcatccaggtcctgccactcctcccaggtgaagtgcacagctacctcctcaaaggacaccaactccagagatttattcttttcttgtagctcttggaaacagccagagaacactggaaacatagccttaaggctgaagaccatcatccagtaccccatctccctcgcggcatcagtgagttcttccctggaaactaggtctcgtataaacttctgcacttcaggccctgcccgcccgcgatgcgcccacgcgtctgctcccacaactggggaacactggtccggccccccgggatcccccgggcccacgggttcctcttcgccctcgcaccgacccgcagggacatagaaccaagccccaggctggcccagctacaagaccgcctctgggtgccgcacttccggagg

SEQ ID NO: 16643 - RNA, 1753 nt, Homo sapiens
  source 1..1753: mol_type = other RNA
gtgttctctgatggacagtgaggaatgacttacagcgaaaggttttcccacattcattgcattcgtagggtttttcccctgtgtgagtccattgatggatagtgaggaatgacttacggtgaaacgttttcccacattcattgcattcatagggtttttcccctgtgtgagttctctgatgtaacctgaggtttgacttattgataaagggttttccacactcattacattcatacggtttttcccctgtgtgtgttctctgatggacagtaagccttgacttatggctaaatgcttcttcacaatggtcacatgcatagggcttttcccctgtgtgagttctatgatgtattgtgaggtatgacttctggctaaaggtttttccacattcactacactgatagggcttttcccctgagtgagttctgtgatgtaaagtgagaagtgacttacagtgaaaagtttttccacattcaatacatttgtagggtttatcccctgtgtgagttctctcatgtaaagtgaggaatgacttacggcgaaaggttttaccacattcattgcatccatagggcttttcccctgtgtgaattctctgatggataatgaggctggacttatagctgaacaatttttcacaccagttacaggcataaggtttttcctcagtaggcatcttgcactgtagcataaggtctgatttgctaatggagggtttctcacattcaacacattcatagggtttctctcctgtgtgtgtctgctgatgtttagtgaagtcagactttctacagcaagttggctgtcctacctgagttatcacttggacaataacagctgagttattacaggctttctcatattcattatatttaccaaaggtctgtactatatgaaccctcttatgtataaagaacattgcctccgtgttgaaggttttcccttgttcattacattgaaaagtctgcagcagagtttgaatcttgtgatgctgagtaagatgttcatgatgtctgtgggatctcctggttatatcacagacatgaggtttctctccagactgtgtctccccaggcttaatagggaaaagcatgttctggcaatcattaaactgcccaggcttcattcctgaactgtttccattatttataatcagatttaaaacatggtttgagttcaaattaaatgtttttcctaattcaactctctcctgagttgatgtgttgctgttggtgattacaatttgccagaaaaatctatcatgactttcatggctcctttcaataaggtcatcaatgatctggacagctgaaagtctcaggtttggggtttcttctactatccatggctctgctccttgctctagcttgaagatcatctcaggtttggtaatgtaatgccccaatgataccaggctgctgtaggtctccagcatcacgtccctgtacagggtcctctgagcatcatccaggtcctgccactcctcccaggtgaagtgcacagctacctcctcaaaggacaccaactccagagatttattcttttcttgtagctcttggaaacagccagagaacactggaaacatagctgcacttcaggccctgcccgcccgcgatgcgcccacgcgtctgctcccacaactggggaacactggtccggccccccgggatcccccgggcccacgggttcctcttcgccctcgcaccgacccgcagggacatagaaccaagccccaggctggcccagctacaag

SEQ ID NO: 16644 - RNA, 1884 nt, Homo sapiens
  source 1..1884: mol_type = other RNA
gtgttctctgatggacagtgaggaatgacttacagcgaaaggttttcccacattcattgcattcgtagggtttttcccctgtgtgagtccattgatggatagtgaggaatgacttacggtgaaacgttttcccacattcattgcattcatagggtttttcccctgtgtgagttctctgatgtaacctgaggtttgacttattgataaagggttttccacactcattacattcatacggtttttcccctgtgtgtgttctctgatggacagtaagccttgacttatggctaaatgcttcttcacaatggtcacatgcatagggcttttcccctgtgtgagttctatgatgtattgtgaggtatgacttctggctaaaggtttttccacattcactacactgatagggcttttcccctgagtgagttctgtgatgtaaagtgagaagtgacttacagtgaaaagtttttccacattcaatacatttgtagggtttatcccctgtgtgagttctctcatgtaaagtgaggaatgacttacggcgaaaggttttaccacattcattgcatccatagggcttttcccctgtgtgaattctctgatggataatgaggctggacttatagctgaacaatttttcacaccagttacaggcataaggtttttcctcagtaggcatcttgcactgtagcataaggtctgatttgctaatggagggtttctcacattcaacacattcatagggtttctctcctgtgtgtgtctgctgatgtttagtgaagtcagactttctacagcaagttggctgtcctacctgagttatcacttggacaataacagctgagttattacaggctttctcatattcattatatttaccaaaggtctgtactatatgaaccctcttatgtataaagaacattgcctccgtgttgaaggttttcccttgttcattacattgaaaagtctgcagcagagtttgaatcttgtgatgctgagtaagatgttcatgatgtctgtgggatctcctggttatatcacagacatgaggtttctctccagactgtgtctccccaggcttaatagggaaaagcatgttctggcaatcattaaactgcccaggcttcattcctgaactgtttccattatttataatcagatttaaaacatggtttgagttcaaattaaatgtttttcctaattcaactctctcctgagttgatgtgttgctgttggtgattacaatttgccagaaaaatctatcatgactttcatggctcctttcaataaggtcatcaatgatctggacagctgaaagtctcaggtttggggtttcttctactatccatggctctgctccttgctctagcttgaagatcatctcaggtttggtaatgtaatgccccaatgataccaggctgctgtaggtctccagcatcacgtccctgtacagggtcctctgagcatcatccaggtcctgccactcctcccaggtgaagtgcacagctacctcctcaaaggacaccaactccagagatttattcttttcttgtagctcttggaaacagccagagaacactggaaacatagctgtgaccttttatcctcctctgaagcaccagtgggaggttagaccagagggctgttctttcaagtgcgcttcttattcatagggaaccctccctttcaaacctgcacttcaggccctgcccgcccgcgatgcgcccacgcgtctgctcccacaactggggaacactggtccggccccccgggatcccccgggcccacgggttcctcttcgccctcgcaccgacccgcagggacatagaaccaagccccaggctggcccagctacaagaccgcctctgggtgccgcacttccggagg

SEQ ID NO: 16645 - RNA, 1806 nt, Homo sapiens
  source 1..1806: mol_type = other RNA
gtgttctctgatggacagtgaggaatgacttacagcgaaaggttttcccacattcattgcattcgtagggtttttcccctgtgtgagtccattgatggatagtgaggaatgacttacggtgaaacgttttcccacattcattgcattcatagggtttttcccctgtgtgagttctctgatgtaacctgaggtttgacttattgataaagggttttccacactcattacattcatacggtttttcccctgtgtgtgttctctgatggacagtaagccttgacttatggctaaatgcttcttcacaatggtcacatgcatagggcttttcccctgtgtgagttctatgatgtattgtgaggtatgacttctggctaaaggtttttccacattcactacactgatagggcttttcccctgagtgagttctgtgatgtaaagtgagaagtgacttacagtgaaaagtttttccacattcaatacatttgtagggtttatcccctgtgtgagttctctcatgtaaagtgaggaatgacttacggcgaaaggttttaccacattcattgcatccatagggcttttcccctgtgtgaattctctgatggataatgaggctggacttatagctgaacaatttttcacaccagttacaggcataaggtttttcctcagtaggcatcttgcactgtagcataaggtctgatttgctaatggagggtttctcacattcaacacattcatagggtttctctcctgtgtgtgtctgctgatgtttagtgaagtcagactttctacagcaagttggctgtcctacctgagttatcacttggacaataacagctgagttattacaggctttctcatattcattatatttaccaaaggtctgtactatatgaaccctcttatgtataaagaacattgcctccgtgttgaaggttttcccttgttcattacattgaaaagtctgcagcagagtttgaatcttgtgatgctgagtaagatgttcatgatgtctgtgggatctcctggttatatcacagacatgaggtttctctccagactgtgtctccccaggcttaatagggaaaagcatgttctggcaatcattaaactgcccaggcttcattcctgaactgtttccattatttataatcagatttaaaacatggtttgagttcaaattaaatgtttttcctaattcaactctctcctgagttgatgtgttgctgttggtgattacaatttgccagaaaaatctatcatgactttcatggctcctttcaataaggtcatcaatgatctggacagctgaaagtctcaggtttggggtttcttctactatccatggctctgctccttgctctagcttgaagatcatctcaggtttggtaatgtaatgccccaatgataccaggctgctgtaggtctccagcatcacgtccctgtacagggtcctctgagcatcatccaggtcctgccactcctcccaggtgaagtgcacagctacctcctcaaaggacaccaactccagagatttattcttttcttgtagctcttggaaacagccagagaacactggaaacatagctgtgaccttttatcctcctctgaagcaccagtgggaggttagaccagagggctgttctttcaagtgcgcttcttattcatagggaaccctccctttcaaaccttataacacacggttaagactgaagtacccttaaggctgaagaccatcatccagtaccccatctccctcgcggcatcagtgagttcttccctggaaactaggtctcgtataaactt

SEQ ID NO: 16646 - RNA, 1782 nt, Homo sapiens
  source 1..1782: mol_type = other RNA
gtgttctctgatggacagtgaggaatgacttacagcgaaaggttttcccacattcattgcattcgtagggtttttcccctgtgtgagtccattgatggatagtgaggaatgacttacggtgaaacgttttcccacattcattgcattcatagggtttttcccctgtgtgagttctctgatgtaacctgaggtttgacttattgataaagggttttccacactcattacattcatacggtttttcccctgtgtgtgttctctgatggacagtaagccttgacttatggctaaatgcttcttcacaatggtcacatgcatagggcttttcccctgtgtgagttctatgatgtattgtgaggtatgacttctggctaaaggtttttccacattcactacactgatagggcttttcccctgagtgagttctgtgatgtaaagtgagaagtgacttacagtgaaaagtttttccacattcaatacatttgtagggtttatcccctgtgtgagttctctcatgtaaagtgaggaatgacttacggcgaaaggttttaccacattcattgcatccatagggcttttcccctgtgtgaattctctgatggataatgaggctggacttatagctgaacaatttttcacaccagttacaggcataaggtttttcctcagtaggcatcttgcactgtagcataaggtctgatttgctaatggagggtttctcacattcaacacattcatagggtttctctcctgtgtgtgtctgctgatgtttagtgaagtcagactttctacagcaagttggctgtcctacctgagttatcacttggacaataacagctgagttattacaggctttctcatattcattatatttaccaaaggtctgtactatatgaaccctcttatgtataaagaacattgcctccgtgttgaaggttttcccttgttcattacattgaaaagtctgcagcagagtttgaatcttgtgatgctgagtaagatgttcatgatgtctgtgggatctcctggttatatcacagacatgaggtttctctccagactgtgtctccccaggcttaatagggaaaagcatgttctggcaatcattaaactgcccaggcttcattcctgaactgtttccattatttataatcagatttaaaacatggtttgagttcaaattaaatgtttttcctaattcaactctctcctgagttgatgtgttgctgttggtgattacaatttgccagaaaaatctatcatgactttcatggctcctttcaataaggtcatcaatgatctggacagctgaaagtctcaggtttggggtttcttctactatccatggctctgctccttgctctagcttgaagatcatctcaggtttggtaatgtaatgccccaatgataccaggctgctgtaggtctccagcatcacgtccctgtacagggtcctctgagcatcatccaggtcctgccactcctcccaggtgaagtgcacagctacctcctcaaaggacaccaactcccttaaggctgaagaccatcatccagtaccccatctccctcgcggcatcagtgagttcttccctggaaactaggtctcgtataaacttctgcacttcaggccctgcccgcccgcgatgcgcccacgcgtctgctcccacaactggggaacactggtccggccccccgggatcccccgggcccacgggttcctcttcgccctcgcaccgacccgcagggacatagaaccaagccccaggctggcccagctacaag

SEQ ID NO: 16647 - RNA, 1852 nt, Homo sapiens
  source 1..1852: mol_type = other RNA
gtgttctctgatggacagtgaggaatgacttacagcgaaaggttttcccacattcattgcattcgtagggtttttcccctgtgtgagtccattgatggatagtgaggaatgacttacggtgaaacgttttcccacattcattgcattcatagggtttttcccctgtgtgagttctctgatgtaacctgaggtttgacttattgataaagggttttccacactcattacattcatacggtttttcccctgtgtgtgttctctgatggacagtaagccttgacttatggctaaatgcttcttcacaatggtcacatgcatagggcttttcccctgtgtgagttctatgatgtattgtgaggtatgacttctggctaaaggtttttccacattcactacactgatagggcttttcccctgagtgagttctgtgatgtaaagtgagaagtgacttacagtgaaaagtttttccacattcaatacatttgtagggtttatcccctgtgtgagttctctcatgtaaagtgaggaatgacttacggcgaaaggttttaccacattcattgcatccatagggcttttcccctgtgtgaattctctgatggataatgaggctggacttatagctgaacaatttttcacaccagttacaggcataaggtttttcctcagtaggcatcttgcactgtagcataaggtctgatttgctaatggagggtttctcacattcaacacattcatagggtttctctcctgtgtgtgtctgctgatgtttagtgaagtcagactttctacagcaagttggctgtcctacctgagttatcacttggacaataacagctgagttattacaggctttctcatattcattatatttaccaaaggtctgtactatatgaaccctcttatgtataaagaacattgcctccgtgttgaaggttttcccttgttcattacattgaaaagtctgcagcagagtttgaatcttgtgatgctgagtaagatgttcatgatgtctgtgggatctcctggttatatcacagacatgaggtttctctccagactgtgtctccccaggcttaatagggaaaagcatgttctggcaatcattaaactgcccaggcttcattcctgaactgtttccattatttataatcagatttaaaacatggtttgagttcaaattaaatgtttttcctaattcaactctctcctgagttgatgtgttgctgttggtgattacaatttgccagaaaaatctatcatgactttcatggctcctttcaataaggtcatcaatgatctggacagctgaaagtctcaggtttggggtttcttctactatccatggctctgctccttgctctagcttgaagatcatctcaggtttggtaatgtaatgccccaatgataccaggctgctgtaggtctccagcatcacgtccctgtacagggtcctctgagcatcatccaggtcctgccactcctcccaggtgaagtgcacagctacctcctcaaaggacaccaactcctgtaatgataccaggctgttgtaggtctccagcatcacgttcctgtacagggtcctctaagcatcatccacgtcctgccactcctcccaggtgaagtgcacagccacatcttcaaaggacaccaaccccagagatttattcttttcttgtagctcttggaaacagccagagaacactggaaacatagctgcacttcaggccctgcccgcccgcgatgcgcccacgcgtctgctcccacaactggggaacactggtccggccccccgggatcccccgggcccacgggttcctcttcgccctcgcaccgacccgcagggacatag

SEQ ID NO: 16648 - RNA, 2511 nt, Homo sapiens
  source 1..2511: mol_type = other RNA
gtgttctctgatggacagtgaggaatgacttacagcgaaaggttttcccacattcattgcattcgtagggtttttcccctgtgtgagtccattgatggatagtgaggaatgacttacggtgaaacgttttcccacattcattgcattcatagggtttttcccctgtgtgagttctctgatgtaacctgaggtttgacttattgataaagggttttccacactcattacattcatacggtttttcccctgtgtgtgttctctgatggacagtaagccttgacttatggctaaatgcttcttcacaatggtcacatgcatagggcttttcccctgtgtgagttctatgatgtattgtgaggtatgacttctggctaaaggtttttccacattcactacactgatagggcttttcccctgagtgagttctgtgatgtaaagtgagaagtgacttacagtgaaaagtttttccacattcaatacatttgtagggtttatcccctgtgtgagttctctcatgtaaagtgaggaatgacttacggcgaaaggttttaccacattcattgcatccatagggcttttcccctgtgtgaattctctgatggataatgaggctggacttatagctgaacaatttttcacaccagttacaggcataaggtttttcctcagtaggcatcttgcactgtagcataaggtctgatttgctaatggagggtttctcacattcaacacattcatagggtttctctcctgtgtgtgtctgctgatgtttagtgaagtcagactttctacagcaagttggctgtcctacctgagttatcacttggacaataacagctgagttattacaggctttctcatattcattatatttaccaaaggtctgtactatatgaaccctcttatgtataaagaacattgcctccgtgttgaaggttttcccttgttcattacattgaaaagtctgcagcagagtttgaatcttgtgatgctgagtaagatgttcatgatgtctgtgggatctcctggttatatcacagacatgaggtttctctccagactgtgtctccccaggcttaatagggaaaagcatgttctggcaatcattaaactgcccaggcttcattcctgaactgtttccattatttataatcagatttaaaacatggtttgagttcaaattaaatgtttttcctaattcaactctctcctgagttgatgtgttgctgttggtgattacaatttgccagaaaaatctatcatgactttcatggctcctttcaataaggtcatcaatgatctggacagctgaaagtctcaggtttggggtttcttctactatccatggctctgctccttgctctagcttgaagatcatctcaggtttggtaatgtaatgccccaatgataccaggctgctgtaggtctccagcatcacgtccctgtacagggtcctctgagcatcatccaggtcctgccactcctcccaggtgaagtgcacagctacctcctcaaaggacaccaactcctgtaatgataccaggctgttgtaggtctccagcatcacgttcctgtacagggtcctctaagcatcatccacgtcctgccactcctcccaggtgaagtgcacagccacatcttcaaaggacaccaaccccagagatttattcttttcttgtagctcttggaaacagccagagaacactggaaacatagctgtgaccttttatcctcctctgaagcaccagtgggaggttagaccagagggctgttctttcaagtgcgcttcttattcatagggaaccctccctttcaaaccttataacacacggttaagactgaagtacccttaaggctgaagaccatcatccagtaccccatctccctcgcggcatcagtgagttcttccctggaaactaggtctcgtataaacttctgtaaacgcaacccaggaggactaggcaggtcacacagtgaaggagggaaccagaaacttcacttgctaaagagacaccgggaaacccaactaatacaaacgcccagtttaagactcgaggcgcacgcgtttcgcactactcctctgggaatggggaacgtctcccgagaactgtgtgttcgcactgggacagatgggcaaactgagcgtcatgcgggttggtaaccggctccctcagcggcaggacaggagcgcggcctgcagactccgggcccagggccaccggcctcgcctacccgctcctgcgcctctagaacccgcttcactgccgggaccccacgcctgtcctcccagcccccgccagggtccgcggcctgcacctgcacttcaggccctgcccgcccgcgatgcgcccacgcgtctgctcccacaactggggaacactggtccggccccccgggatcccccgggcccacgggttcctcttcgccctcgcaccgacccgcagggacatagaaccaagccccaggctggcccagctacaagaccgcctctgggtgccgcacttccggagg

SEQ ID NO: 16649 - RNA, 401 nt, Homo sapiens
  source 1..401: mol_type = other RNA
gttagggccaacatctcttgggaaaggctgtctctgattctctggaattaaaatgggagataccacaatggacctcttttgtcttgggacaggagaagttcttgcaaatttaaatatatcagtttagaattgactggtcctcaatgaattcagctggctgattgatatggaacactttctgctgaaatccaggagtgcagtccaaatcttctgcagatgttagcagcagcacctgggacaggagaacgcacagaacgagcggagttctcggctgcattttgtccgactagaagcgcccggcggcgttttcattcatgcacgcggctgcactgagcatattttccgtgggagccaggctttgaggagaggctctgcctcgccagccagccaacttcccaaat

SEQ ID NO: 16650 - RNA, 716 nt, Homo sapiens
  source 1..716: mol_type = other RNA
gttagggccaacatctcttgggaaaggctgtctctgattctctggaattaaaatgggagataccacaatggacctcttttgtcttgggacaggagaagttcttgcaaatttaaatatatcctgcaaggagccctggatgtctttccccccgacaatcacgagttctgccatatcttccgcatggggggtccgtgcatggacgaacagagttttgcccactgcagttatgtttctcagagcaactaagccgccatcgctgttcaccttgaagtatgggctcgagacctcatagcgtagcttgtcgtttcccttacagtcactgaaggtcaagtttagaattgactggtcctcaatgaattcagctggctgattgatatggaacactttctgctgaaatccaggagtgcagtccaaatcttctgcagatgttagcagcagcacctgcatggttgaagctgcaggtgggtcacgcccaggcatctgtgggccattctcactgggatgttcttgctgggggaaccatgcagtgcaggtgggttgtttggccctgggacaggagaacgcacagaacgagcggagttctcggctgcattttgtccgactagaagcgcccggcggcgttttcattcatgcacgcggctgcactgagcatattttccgtgggagccaggctttgaggagaggctctgcctcgccagccagccaacttcccaaat

SEQ ID NO: 16651 - RNA, 810 nt, Homo sapiens
  source 1..810: mol_type = other RNA
gttagggccaacatctcttgggaaaggctgtctctgattctctggaattaaaatgggagataccacaatggacctcttttgtcttgggacaggagaagttcttgcaaatttaaatatatcctgcaaggagccctggatgtctttccccccgacaatcacgagttctgccatatcttccgcatggggggtccgtgcatggacgaacagagttttgcccactgcagttatgtttctcagagcaactaagccgccatcgctgttcaccttgaagtatgggctcgagacctcatagcgtagcttgtcgtttcccttacagtcactgaaggtcaagtttagaattgactggtcctcaatgaattcagctggctgattgatatggaacactttctgctgaaatccaggagtgcagtccaaatcttctgcagatgttagcagcagcacctgcatggttgaagctgcaggtgggtcacgcccaggcatctgtgggccattctcactgggatgttcttgctgggggaaccatgcagtgcaggtgggttgtttggccctgggacaggagaacgcacagaacgagcggagttctcggctgcattttgtccgactagaagcgcccggcggcgttttcattcatgcacgcggctgcactgagcatattttccgtgggagccaggctttgaggagaggctctgcctcgccagccagccaacttcccaaatagatcagcagcagcatcacgaaagcattgggtagaggctgatgaccaggaccaatggctttacaagacggattccttcctaacgctccctcgtt

SEQ ID NO: 16652 - RNA, 862 nt, Homo sapiens
  source 1..862: mol_type = other RNA
gttagggccaacatctcttgggaaaggctgtctctgattctctggaattaaaatgggagataccacaatggacctcttttgtcttgggacaggagaagttcttgcaaatttaaatatatcctgcaaggagccctggatgtctttccccccgacaatcacgagttctgccatatcttccgcatggggggtccgtgcatggacgaacagagttttgcccactgcagttatgtttctcagagcaactaagccgccatcgctgttcaccttgaagtatgggctcgagacctcatagcgtagcttgtcgtttcccttacagtcactgaaggtcaagtttagaattgactggtcctcaatgaattcagctggctgattgatatggaacactttctgctgaaatccaggagtgcagtccaaatcttctgcagatgttagcagcagcacctgcatggttgaagctgcaggtgggtcacgcccaggcatctgtgggccattctcactgggatgttcttgctgggggaaccatgcagtgcaggtgggttgtttggccctgggacaggagaacgcacagaacgagcggagttctcggctgcattttgtccgactagaagcgcccggcggcgttttcattcatgcacgcggctgcactgagcatattttccgtgggagccaggctttgaggagaggctctgcctcgccagccagccaacttcccaaatagatcagcagcagcatcacgaaagcattgggtagaggctgatgaccaggaccaatggctttacaagacggattccttcctaacgctccctcgttttgcatggcagatacggggtgagcacctcgcgaggagcgagccccgcggagg

SEQ ID NO: 16653 - RNA, 610 nt, Homo sapiens
  source 1..610: mol_type = other RNA
gttagggccaacatctcttgggaaaggctgtctctgattctctggaattaaaatgggagataccacaatggacctcttttgtcttgggacaggagaagttcttgcaaatttaaatatatcctgcaaggagccctggatgtctttccccccgacaatcacgagttctgccatatcttccgcatggggggtccgtgcatggacgaacagagttttgcccactgcagttatgtttctcagagcaactaagccgccatcgctgttcaccttgaagtatgggctcgagacctcatagcgtagcttgtcgtttcccttacagtcactgaaggtcaagtttagaattgactggtcctcaatgaattcagctggctgattgatatggaacactttctgctgaaatccaggagtgcagtccaaatcttctgcagatgttagcagcagcacctgggacaggagaacgcacagaacgagcggagttctcggctgcattttgtccgactagaagcgcccggcggcgttttcattcatgcacgcggctgcactgagcatattttccgtgggagccaggctttgaggagaggctctgcctcgccagccagccaacttcccaaat

SEQ ID NO: 16654 - RNA, 395 nt, Homo sapiens
  source 1..395: mol_type = other RNA
gttagggccaacatctcttgggaaaggctgtctctgattctctggaattaaaatgggagataccacaatggacctcttttgtcttgggacaggagaagttcttgcaaatttaaatatatccttattggcttgctcaacattcgccaaaccctgaacgtcatcacacaagtgagagggtagcatatttcatatgtgactagtctccaaagttacagagtcttgggaagttccacttaatagccaagcagcaatgagtcagtcagttttcctccataagcctcagttattaccacaacatcagtatgggaacatcattaatgttttcttcctgtgtggtcaggggagctcaggagtggagattggcccctaaagtccagccctcaccagctatgcca

SEQ ID NO: 16655 - RNA, 3623 nt, Homo sapiens
  source 1..3623: mol_type = other RNA
gttagggccaacatctcttggttcagccactaaacttgagcataaagtcaatgtctcttccttcacccaccctcccacccatccacccccatgcaaggctgattcagtcttaaccttgtctcaaaagggttacgggaaattccatccatcccagaacaagtaggttaatttcactgagtaacaagttttttgttctttcttgtgggttggtttctgtggtttgagccagcaaaactcttaaatggagaataagataagataaaaaacagatacgagagtagaactttctgctttcaattggcatctctgtatccaaggccagagcctttctgtggtggaaaagtgacaaaggccttagcgaatggcagagaaaagccacccttgtcagaacaccttggactccaagccttcgcacacagtgtcagaaaaatcaaaaagaaaagaaaaaaaggtaattaaagattctgccctcttccttctgggtttccttttgcttatttaacttaatctacccaagtaaagctgatccagagagagctctgttcgcctgctcacccccattctcactctccagcacagtattgctcgtgtggttggctgcaccttgtccgcgaagcacccgcggagaacgtctggatttggacgcgcgcctgcctcctggcttccgtcaccacagcggcgcgggtccctccgacgccccgtagagctcggccagcttccggaagcggggcccccagtccgtcaggaagtcgaagctctgttccgagtccgacgtggccgactgcagggagctcagcgaccccgccacagagccgtccccctcgaacatatacgtctggagggagtcgaagggcggtgcccacaggtccatgtcggcctcgtagagcttggccagcacgtagctgtggacagtgctgttcactgcgcacgtctgaggcacgtagcgggagaggctctcgatctcgggcagcatgtcctgccgcgtcttgggggcggcccccgcctgcgcctcccgggggttccacatggccgcgatgtcgaaggcctcggtgtcctcctcgccgccgccctcgtcgtcgtagcggacgatgttctcgtggatgttttcctcgtcgtcgatgatgtatggttgtttccggtgccgcctcatggacaaaatgagcaacaccagcactaagaggacaaagatgcaggcgaggatggcaatgagggcgccccggctcaaactgactgggagcatgtaggcctctgggctgcaggacatgacgtggccgtcgtcatcacagctgcacacttggatggtcagtgtgcctgtgctgctcagcacgggctgcccgctatctgctatcaggataggcaggtgaaagacactctgctcctgctgccggaaaccagacctcctggttagaatccgtgctgtgttatcttggttgtcccttatggtaaagttggggttgttagcagcctcaggagccaagctgtagtagaaatgctgaccattgcgtgggtcatcttggtccaccgcactcactgtctggatcagctgtcctgccttggcgttctcacagacaaaagcttcatagaatctggggaactctggagcattgtcattcacatctaagactttgattgtgacaggaacacttccaacctgggagggattgttcatttccatagcaaggacagtgatattatgccaagaaaattcttcccggtctaggggtcttgctgtcattagggcacctgttgtaatgtcaacatagaaaaatcttccagggtcactgcttctatcaatggagtatctgattgagttgttggtcacatctgggtccttggcagaaatgatctgtatggttgttccaatcgccacatcctcaggcacctccacaaagtaaaagccaggttcaaacacagggggctcgtccacgtcttccacactgatgtgcactgttgttgtgtcctgaaatgggcccaagttcagaaaacgcatctctaggtgaggattggctccctccacctttaaggtgtagcttttcttgctttcaaaactcaggggcttcttcacagttatgataccaacttggaaattgggatctgtgctaatgtcaaaggcatctgcaccatctccatccacaatagtatatttcatctctgcattgatgccttcatccaagtccttggcaaacactctcccgacagtggagctaattggagctgattccaacacactcatctggtaatgtttctggggaaagcggggtgggttatcattgacatctgagagggtgatgttgactgttgtggtcccagctaatcctccaagctgccctcccatgtccttggcttggataatcacttcgtagtattctttggcttctctgtccatgttcatgagcgctgtcctaattacacctgttttagagtccacagaaaaatatggctggccctgaagaatgctgtacaccaccctggcactgttgccgtaggtcgggtcatctgcatctgtggctgtcacttggatgacggaggtacccacaggggacatttctggcacagtggccacataaggtccgtccaggaacttgggctcattgtcattgatgtcttgaattttgatgatgaactctgactcgggctccattggcctgcccgtccgcctgtctagggcttgagcccttagagtatactgggctctttcctctcggtcgagcctctgaatggcgtggatgtctccagtggtgtcgtcgatggtaaacacgatgccagcaccttctcccgagaggatgtatttgatggatccgtctcccctgtccatatctgaatgaagcttgccgacatacaaagggtcggtcccagtgtactcttccagaacgaaaaactggttccaaacccagctcctcttggtccgctgatgtgactgtggcttgtctgacaggagtgcttctaattcaccttgtggtgttggggtgtccgagagaacggtggtcgtaaggtccatcagcccccagaagtacaaggacatgccaagtccaagccagttctttgcattgctcattctaccagaagtccacatgggattgccaggttttcagaaaatgaaggagaatgataagcaactggaacttgagtattttccaaatttaaaaaaatacacagtttttgattggacacttatgcttcctaaatgagatcccgtttcaagtcaatctgcttgaagttgacttcctggcaccgccggcgactctccggagaccttcggtcctaactgctccagggcgggcgttctgctcacgtagctgcctcccccactgggcggctggtgccccgctgggtctcttcacccctgctcgcggcgctgtccccgccccccacccccctaccccctctgtcagaagtgtcacagcttttctgccttcggatgtttcgcaaagtctccgtgcggttgccaggagttggggggtactgccaagtgcaccaaccccgccgatgccctgccctgccctcccgcggccaccgcgttcggcctgtccagtgagaagagccccctggtcgcggtcaccgtcccccgagcgtggcgcgcggtccgcttcccctccctcgcgccttccctagcaggagtggct

SEQ ID NO: 16656 - RNA, 9425 nt, Homo sapiens
  source 1..9425: mol_type = other RNA
gttagggccaacatctcttggttcagccactaaacttgagcataaagtcaatgtctcttccttcacccaccctcccacccatccacccccatgcaaggctgattcagtcttaaccttgtctcaaaagggttacgggaaattccatccatcccagaacaagtaggttaatttcactgagtaacaagttttttgttctttcttgtgggttggtttctgtggtttgagccagcaaaactcttaaatggagaataagataagataaaaaacagatacgagagtagaactttctgctttcaattggcatctctgtatccaaggccagagcctttctgtggtggaaaagtgacaaaggccttagcgaatggcagagaaaagccacccttgtcagaacaccttggactccaagccttcgcacacagtgtcagaaaaatcaaaaagaaaagaaaaaaaggtaattaaagattctgccctcttccttctgggtttccttttgcttatttaacttaatctacccaagtaaagctgatccagagagagctctgttcgcctgctcacccccattctcactctccagcacagtattgctcgtgtggttggctgcaccttgtccgcgaagcacccgcggagaacgtctggatttggacgcgcgcctgcctcctggcttccgtcaccacagcggcgcgggtccctccgacgccccgtagagctcggccagcttccggaagcggggcccccagtccgtcaggaagtcgaagctctgttccgagtccgacgtggccgactgcagggagctcagcgaccccgccacagagccgtccccctcgaacatatacgtctggagggagtcgaagggcggtgcccacaggtccatgtcggcctcgtagagcttggccagcacgtagctgtggacagtgctgttcactgcgcacgtctgaggcacgtagcgggagaggctctcgatctcgggcagcatgtcctgccgcgtcttgggggcggcccccgcctgcgcctcccgggggttccacatggccgcgatgtcgaaggcctcggtgtcctcctcgccgccgccctcgtcgtcgtagcggacgatgttctcgtggatgttttcctcgtcgtcgatgatgtatggttgtttccggtgccgcctcatggacaaaatgagcaacaccagcactaagaggacaaagatgcaggcgaggatggcaatgagggcgccccggctcaaactgactgggagcatgtaggcctctgggctgcaggacatgacgtggccgtcgtcatcacagctgcacacttggatggtcagtgtgcctgtgctgctcagcacgggctgcccgctatctgctatcaggataggcaggtgaaagacactctgctcctgctgccggaaaccagacctcctggttagaatccgtgctgtgttatcttggttgtcccttatggtaaagttggggttgttagcagcctcaggagccaagctgtagtagaaatgctgaccattgcgtgggtcatcttggtccaccgcactcactgtctggatcagctgtcctgccttggcgttctcacagacaaaagcttcatagaatctggggaactctggagcattgtcattcacatctaagactttgattgtgacaggaacacttccaacctgggagggattgttcatttccatagcaaggacagtgatattatgccaagaaaattcttcccggtctaggggtcttgctgtcattagggcacctgttgtaatgtcaacatagaaaaatcttccagggtcactgcttctatcaatggagtatctgattgagttgttggtcacatctgggtccttggcagaaatgatctgtatggttgttccaatcgccacatcctcaggcacctccacaaagtaaaagccaggttcaaacacagggggctcgtccacgtcttccacactgatgtgcactgttgttgtgtcctgaaatgggcccaagttcagaaaacgcatctctaggtgaggattggctccctccacctttaaggtgtagcttttcttgctttcaaaactcaggggcttcttcacagttatgataccaacttggaaattgggatctgtgctaatgtcaaaggcatctgcaccatctccatccacaatagtatatttcatctctgcattgatgccttcatccaagtccttggcaaacactctcccgacagtggagctaattggagctgattccaacacactcatctggtaatgtttctggggaaagcggggtgggttatcattgacatctgagagggtgatgttgactgttgtggtcccagctaatcctccaagctgccctcccatgtccttggcttggataatcacttcgtagtattctttggcttctctgtccatgttcatgagcgctgtcctaattacacctgttttagagtccacagaaaaatatggctggccctgaagaatgctgtacaccaccctggcactgttgccgtaggtcgggtcatctgcatctgtggctgtcacttggatgacggaggtacccacaggggacatttctggcacagtggccacataaggtccgtccaggaacttgggctcattgtcattgatgtcttgaattttgatgatgaactctgactcgggctccattggcctgcccgtccgcctgtctagggcttgagcccttagagtatactgggctctttcctctcggtcgagcctctgaatggcgtggatgtctccagtggtgtcgtcgatggtaaacacgatgccagcaccttctcccgagaggatgtatttgatggatccgtctcccctgtccatatctgaatgaagcttgccgacatacaaagggtcggtcccagtgtactcttccagaacgaaaaactggttccaaacccagctcctcttggtccgctgatgtgactgtggcttgtctgacaggagtgcttctaattcaccttgtggtgttggggtgtccgagagaacggtggtcgtaaggtccatcagcccccagaagtacaaggacatgccaagtccaagccagttctttgcattgctcattctaccagaagtccacatgggattgccaggttttcagaaaatgaaggagaatgataagcaactggaacttgagtattttccaaatttaaaaaaatacacagtttttgattggacacttatgcttcctaaatgagatcccgtttcaagtcaatctgcttgaagttgacttcttttctcctttcacggagtgcgctatttttgcattttcccgagcttgcccctgagtggtggagttcccttcctgctgccagctcccactgtatgtcaggacaacttaaagtggccctccttttgccagttccagattagtctttaaattagaatcagggatgaaagaggccatcggatgcgaggacatcagcccagtaactttgagggaagaaggttttccttcccctgctgcctatgccgtggggtttgagcacgtctctcggggggaagtaagacccagccagcccccaagttgctgatgcagcctaaagcgacttaggaagggagtgggaacaaaaggcatctcttaagttaggtgattagcagcaaatgatgtatgggggtgggagggagcctggtatacaaggaaggggagctggcagttgcccttgtctggagggggaaggacaaagaatgctggccctgaacatttgaggccctgggggatttcttaacggaatcaaacagcacaggactatgtgcagccttgtacagtaagagctaaagttctttggacatgttgtcctcacagacagctgaaaatatctagtggcaaatacctatcagctactgatgcatttcagaaacaaaagataatgggaaggctaacaaatcacatgtctttttcacttaccattacttagtgtttccagtaagtaaatgcagtatctcagctgagcttctctttcaaattattgttaattaaataatactccctaagaaacctgtcattaccgacagccaggaatgggtttgttgagtttgcctgaggctataaatgctccgacaaacgggatcttaattgccataagaggtaatatcattggggattgtagttcactttttccaacaattttatagtatgttttacatcttaaacttttgcattttgcttctacgtgtggagttccacagggccacagggatcattctctaatgattcatccattgaataagccattcttcataatggaaaaaatgcatgttgctattgaatctgtaatttccccccagttccattatgactaaagagaagcaattgataacagattttaaaattaacttaatttcctccagttcattatattacttatcctttgaaataaatgacttttgctgggagatataatttctggtatgtcacggacctaactctgacattatctcttgtcaactgttttcctagtagacaggagagttaggtaggtggaacaattatcactggatggagttgaaagggagacagatgagggcatttggctgcagagagcaacatgtgctatggcctagaatttaaagtgaccttatctacaaacattttccttctgttcatgagcagagaataaggacaagtattaagaaaaagtcacatttttttcagagttataaaagtctccatatgccatttcaaaaagaagtactatttcagccttttcttaaatgacctctttttcatcataatataatatatttctttcaccttttgactggtactttggtttcttaatcaagttacatgtttcagaaaaattacactttagaatgcgtcttggtggtatttcattccaacagtttcatttggttgaattaatgtgcagctgtggcttagtggagggagagagagggagggagggagagaaagaggagaagatagaagaaggctcatataatccaacctccaagcataactttcctcaatttcacgtttcagtatcattatagaaacctctatctgtaataaaagcataatttaggtcaatagtactaaaacgtatatacccatattatatcagtgatctactgttctgtggtcaaaattctttcctttcttcctcttcaccaagttcacctcttgtttttgtcctttctctatctggtgtcacttgataatctttcattctcttttttttttctttccaggttcttgtctctttttcccgttaaggcgtgaatgagcaggcatctcagccaatatgtctatacatggctgaatacacttggtgaaaagcagggtctccttttgtctggaccctggatggctgcgtgtcattccgcaccaacgggcagggcctccctcacagtaggaactttgcaataattgccagaacaaattgagctcaggcttatcggttcctttcctttttccgttggaaaatggagggaataggggaacaaggccagttttgaccattaacaatacggcgtagaaatagattggatacagccagtgcccagtcttgttgcaaacagtcacgggataggttgtgtacagggatgataagatgcgaccctgtaatcacacagctaaccgagccctgatttctccacaccccccagggtgctctggtgtgtatgatacgcatttatagccgttggcaggggaattgttggaactgacacacagaccgccggcagaggtgagaacaaaagatgtgatgggttggtgcttgtgttctttttgcatctggtgaagaccagcagaggcaactctcaaactgttttcaccagattgcaatgagaaaaatggtctttggtaagaaatctgaacatataggggaaagaaactcatttaaaaatcatgttacactttctttttttccctgtacaagtctttatcagaatctctatgaatcattgatatagttcatgtacctacatccctctccccgtgttcggtgtagtaagcatgtgtgtatgtatgtgtatgtgtaactaacattttttgttaatttcatgtgtatataggtaactggaaatgataatgtatatacataaatgtaaatgcaaacatgcaatggcatgggtgattttctctttacatacatacgtatgtttatactccaaaggttgattctaaatctacaaaatgccacaagctccctgctagaaatctttccttaatgagatattgtgttggatttgcttgagggtcacatacacaaccaaggttgtatcctgtgttgcccactataggatggttgagaggggagaggagacaaggccttaccctaactgggcagccagactgttgtttcgaaactgctgaagcagccagatcacctgtgtgtgtgacaacccagtctgtatttctaaaataatgttatttatataggggtgtgtgtgtgtgtgtgtgtgtgtgtgtgtgtgtgtgtgtattcattctcatccaactggggttaagctttgctcagctgctttcaaagtgactggaagtagacgacatgaggagctacagccaactgagtggctttccatctgcctctgctttgcttggaaataaccagccagagcaatggttttagctttattcatttgttgttgttgttctgatctgaagcagaggctgacatgaaacaaacatagcatttccttttgaaaattgaattctgaagttggcttcatctttccagaatcacagtgctattgcagttccttcctagctttgtgaatgtcataaacaatttgcatataaagctccaaatgtggaggtaatgaccacatttgtgttttaggatttttgaggggaggggtttgatttttagtggttatgaagggatttgttgagatttgtgggatgaatggaactagtttcccctatacaggagagatcaagaaatggggaaacaaattcataataaagaacacctttgccagtcttttactggcaatttttaaggaaacacagcaaaatgtaaagtcatacaaatgtggctttttgaggaacttcattagcatcacccacaatccatagtttacaataaatgggcactggggcccccacaggtcatggcccatagccagcttgctgcaatggaagcgatgcttacagtaaggcgagttccctggacacgatatatgaggtatggatgacagtacattatctaagccagttgcactgtagtgacttgaaattggaagacacttagtggagcaagtaggggggaaaaagggatactagagaaacacagtgcattaaaagtctctcagcattaaatatgcttaggagagataagaaaaagaatattcttagaaaagatttaccattattctttagcagtatgtccttcccctccccaaacacacacactcacacacctacacatccctacagacagaaatgaaaagggatttccttcactcagaacatccttagcgtatcttgatgtcttgaatcttttggggccataaagaaaaatacttgttttagggagaaataaggatttgagaatcttggctatcaagattgtcatttctgttctccacacatgcagtgaaaggcaaaccatgcaattttgacttaatttcattttgacgctggtgattggatcacggctgctcttgcagatacagttgaggcctattaacttgagagtaatcacaaagggacccgtgatatgtacagaatcacattctccaggggagacaacttgatgggaagtatggctgcattgcctgggttctaacctctgctccactgtgtacaggatgtgtaaacttgggcaagtacttaacctctttgtgcatccgagtccacacctgtaaaacgaagctaatagtagttcctatgtctactacataagtcactatatgtgaggtaatggggcagagccttcgcacacagcaaatgctcaatagatactagttattagtactagtaagcgaacgtaagccttggggtcaggcagaatcagctttagattctacttctgtgttttttggcaaatgatttaatatttctgaggcccagacggtttccaatgcatagaattgcagggttgctataagcatgaaatcctcttgtgtgccacaggaaggccccgtgtgtagaacataagagatgctcagtaaaagtttgtctttccaaaagtagagaagaaaatatccctatggcataaactatcatgttcatctttcctcataattgtttggatcttttccttcattatttttggagggagggagtgaatttttctaacttgggatttcatggtagttattggccaggagtggtggttcctcaaagtgattgaagttgcaaactctgtatttgatggatagtgagaaatggaagcttgttagtaatgagacataaaattgtaactggcttgtcaaaaagacactctatacctgacttttggggaaaaaaaccccaaacaccataaatatgtttcttcattgtgatgatgtggaaattgtcagattctcaagcggagaagaaggcaaattaggcctcacaagcctctccaaatacagagagaataggaaactgattttccaatactacaatttgcacatgattctaatgagaaaatctgaggggatatcatggcaatatgtctccccagtggcagctgatcattatatatatatatactgtcattagagatggtaccagacacctttaggagtgtctgtctagcatatttctgtcttagaactgaccttccatccttaaaggactggcccctgcagccttgtttgtaacaaagaacttgcccatcccccaggctgaaactggaacaggatggacactgagccaagccaggccaagcacattgtttgctgggagtatggaagggaacctgcaaggatggctggggcgctgtgccctgcagaagcagagcagaggaagtgggacagagaagagggaggcggggagggcatgggaagagggcaggctcttgctccttgtttcagtccctctggaggctgagcccaaactcctgtgtgtggattctgagttacctctgtagttgtgcgctaatttctttctttgccttaaagccatcttgagggaatgttgtttccctcagacctaaactttactaggaggagttcccaaaactttactaggttagtccctagatagatacctcatgggaagctggcctcaagttgtggatccaaggaaaaaccattgagagatttccatggacttaatcctcttctctgtcccctagattgtttcgaacacctttattaattaggtgaactgtggaaggtaaagtcgtaacaagacggcccttgaagaaatggtggtgacatcatgagctgcatgtcccgtaactctgcgtgactagaacatcatgtcatgaaaggatttttgaatactcatttttaaagaaatgcagtatgatatagcatttaagtaaaatagtaa

SEQ ID NO: 16657 - RNA, 39 nt, Homo sapiens
  source 1..39: mol_type = other RNA
gttcaaatccagatctataacctgtgtgactttaggcaa

SEQ ID NO: 16658 - RNA, 69 nt, Homo sapiens
  source 1..69: mol_type = other RNA
gttcctgctgaactgagccagtgtacacaaaccaactgtgtttcagctcagtaggcacgggaggcagag

SEQ ID NO: 16659 - RNA, 6628 nt, Homo sapiens
  source 1..6628: mol_type = other RNA
gttcctgctgaactgagccagtgtacacaaaccaactgtgtttcagctcagtaggcacgggaggcagagcccagggaggccaggcagcaggatggcaggcagacaggcggcagcaggggacaggcggcaaggccagaggaggtgagggcctggggggcggaacttagccactgtgaacacgacttggtgtggaccctgctcacaagcagctaagccctgctcctcaggccaggcacaggcttcggggcctctctgccaccccgtccccgggcagcatcctcggtggcagagctcagggtcggttggaaatccctggcaatgtgatttgtgacaggaagcaaatcccatccccaggaaccccagccggccgtggcacaggggtgaggggggcaccgggcggggccagaggctggcacctggaggggagaaagagagagagagcaaaggaggtaatgagatttggggacacctcccctccaggtccccagatgcttcctttgatcacagggaagctcttttctcatatgcaggagccaccacacggggagctggagcctagctgtgccctccgttccagccccaggactggagaggcagagatacctagagggcccatgcgggacaaggaggctacagcaacttgcatggccaagctcccccctcattgagccctgggcaggccaaatggggccatggggagaggaagccaaggggggccaggcaggcgggtgaggaagtgatctcaccccagctggcgccacttcctagaagcctggagggcaggaggaaaccaccagggcctccccccccgtggcccggtctcctcagtggccagggcttagcccacacccaccagggcggatgccggcagcaaggcacccccctctctttctagacacgcaccccccgccccccagagcacaggatccaagctccaagatacaggcctctccacccaaacagcccaaggttcaaatccttgctccacagtttcccaaagactctccaaagcttcagtttccccatctgtaaaatggagccaagagcctcttttgcatagcccagtgagatgtcaccgagtatgtatgtcactcagtaagtgcccagcaccagggcaagatacaggattttcaggacccggtgcaaaatgaacacgtggtcctctagttcgaaaactaagaatttcaggccaagcatggcggctcacgcctgtaatcccagcactttgggaggccgaggcaggagagtcacctgaggccaggagttcaagaccagcctgcgcaatacgacaataccccatctctacaaaaaaaaaaaatattttttcttttttgagacagggtctcactctgtcgccacggctagagtgcaggggtgcaatcacagctcactgcagcctcagcctcccaggttcaagtgatcctcccaccttagcctccggggtagctgggactacagctatgcaccaccatgcccggctaattttttctttttcttttctttttttttttttttgagacagagtctcgccctgtcgcccaggctggagtgcaatggcgtgatctcggttcactgcaacctccacctccagagttcaagcaattctcctgcttcagcctcccgagtagctgggattacaggtgcccgccaccacgcccagttaagttttgtatttttagtagagacggggtttcaccatgttggccaggctggtctcgacctcctgacctcaggtgatccgcccacctcggctttccaaagtgctgggattacaggcgtgagccaccacacctggccctaatttttgtagagatggggttttgccatgttgcccagactggtctccaactcctgggctcaagcaatccgcctgcctcagcctcccaaagtgctgggcttacaggcctgagccacagtgtctggcccacaaaaaattcactaaaaaatcagccaggagtggtggtacacatctgtagccccagctactcaggcggctgaggtgggaggactgcttgagcccaggagtttgaggctgccgtgatctatgaccatgccactgaactccagcctaagtgacagagcaagaccctatctctaaaataaacaaaaacaagtttaaaaaaagaaaataatttcaggctgagcgcggtggctcatccctataatcccggcacttcgggaggccaagacaggaagatcgcttggggccaggagttcgagaccagcctgggcaatacaagacaaaaaaattaataataataaaaaaaaattcatgaccccagcagtgcaacattaaactaacctccaggtccctccaagcagggctgccgtgagactgcccgtttcacaaatgcatgaagccagccctaagtctttagtgagtggagcttcttttgataagagcccaacacctggctagcagactccagttttggagcccaagtctgcccagatttgaaagccccagctctgcagcttctgagctgggtgactctgggcaagtcactcaacctctctgggcctcagcttccccatctgcaaaacagggataataagtatggacttcataagtcatggtgaggaccccatgagtgataaacatgatcacgacagagctgctgctgtctttgccaaggcaaaggataacggaaacgtgggtgtctcacaccaggaccccagtgtccgcccgatgtggtggcgctcaccacttcgagacaggcggcgagtgatgtcctgttttgtcccctccctatacacacatacacacataccagccactctttcccatcaggccccagcccagccctgtccccttagggtctggaggcgccaactgggagcaggcgaggccccgcagggcggccagcctccctgggccgcctccggaagtgagacagcacattcgtgtcccagggacgagaacgggaagggcggccatttggccaggctcgtttcctgtggggtttcccctgcacagagcccagggccggggccaaggccactccccatccccgcaggcacaaaaggtctgggtcttgagtggaaggggtgctgccatgcaggtgcccaggagacagggtcccctttaccaatcatggtgcacttctcaggctcttgggagatggtgtccagggggaaaccaagctcctagcagctggaggcatgagggagagggcgggcccctgggctggggagcaaagcaggccccaggctgcatcaggacaccccggccagccaatgcatgtgggtatgcctgaataccccctccagacagcgtgtgcgtggaccagacacacaagggtatgtatgtgtaccgctacccccccaaccccatgctccaagaatgaatcaggggcagcttccgccgggggcgccaccaccacctccgcccccaagcctggtccccaaatactttccaccctcacagagcagctgggatcggaaaataccaagggctgcaggccccgccctgcccgccgcgccacccgccctcccagcctgtcactaacgctttgcctaatgggcccagactctcagcagaagctccgtgggctgggcctcgagccagccgccaacctgggctgcccggccaagcgccgcctgaccaggagccccccgcccctctgccccaatcccagtgcagcgacaataacaaccgccccgatgggcagccctcagagggtggcactgggtagggaaagtcagggcactgacaagtgggtgggccccgctgcccacccagggctggggtggggggaggctcaggaaggggtgagtaagtgagggctgaatcacttgttataaataggggaaccatgaaagtgacatcccagcccccattgcgtcccgccagtccacactctaacccccacttagactttaatctttcccagaccaatcacagaattcccaggggccccctcaccttcatgttgggaacccttagtagagtggtacaccccgtcatcaggtccacccctgccttctccccacataggtacattttgcagtgagggcctggctgtgggggtcccctggccttgaatgcagtcactggtgtctgcgccctatccacctccctcaacgcaccgattcccaggcccaaggctcagggcctctaggctctccaaggcattctcagggtgtgggccaccacagtcctggagggtgaccccagaacctaggccaggcgggaggccagggggcttggcatcttcgaagtcagttccccaggcaccgaggccccacatcctagaccacccagccctgctctgcccagggccacagctcagtgaccacacccagggtggcgccagctccagcaccctggggcaaggcgtcgctggagcgtgactcagccgtgcccagcatggcggcgcccttctctgcccagggattctcacccacacccactgccctccgctcaacatccttcccaggcgaccggccctaaaggacacaccttccccagacacacctccgtgtccacccaggacaccaggagggaagaaggcggccaggggcaaagtgtacacttctctccgtcccatttccaaatgcttcccatttatagatagaataattaaggctcagagattcagactggggcttaaggtcatggaataagtcttaaaaaaaaaaaaaaaaaaaagccaggcctgactgtggcctaaaacacatccaacgtggaaaacagaggttacaggaaggagttttctcaagatcgcccaaggttcctggcgccgttattcatggaggacagaatcccccacccagctttccaaggtgaagggcaaactccaaaaaatgctttaagaggtatcaaagcaccacctagatcgggcgagcgggtcaccccagtgtacccaccgggctaattaccctgggattgcagatagatgggggcctgccccgcagctgcggtctgcatggaacatctggcgtccacttgcattgttagagggtgggcacgacacgggggtccctcctaaagcatccgcctctgctgtctttctccagcgagcaagggtcggcggaggctcagtggccaggccagcacagacaggcccgaccctctggacacgccctgtcacgcatgtgctccgcgtgccagccccaggccaggccggcacctattttagggccccctctagatccacaggcaaggcctgcctgttggggtcttgaaggagctcccagaggacgtgctgcaagggcagagggccatgggtgcctcacgggatcagagaacaaagctagcaccagccccagggcctgtgccttcccaggacatcggcatgtgaacacatgtacccaggctggcccgggcagggcatgtgggcgagcggacagggtgtgtccaacatcacctcgcctctaagcctgggcacctgttgggtacagccctccagctggggcaggactgccagaggacaccccttatgccaggggtcccccagcccccagcctcaccctcatagaccaggagtcagaggctgccagctggggaaggttgggaagggggcaggtgacaaggagccagctgcacagccaaaacattcaagaagccactgggtctggggcctggctgggctgggctgggctgggctgggcaggaaggtcagttagggctaagggctttaggggcagccaaatctagtgctaaaatcagaaaacagtctggggctaagacagaggggtcggggttcagtctgggcccttttaacctcctccttcagccaaaaggcacggggaccccaagctgcacagggctggtccccaacctggctttccttcctatgcaaccttgaatgagcgcttttctccgaagggaaaggagacatccccccagctcccaccagcccctgcccaacaagagaccttccccctacccagcgggcgacacgtcaagaacttggaccggtatccacccccgcccccacccaaagaactctgagagacccccccaacccattcctcccgtccaaaggccaggtcggggggctaggagtggggtaggcatatgcatatccaagcccctcaacccaagccccatgtccgagccggacacaagccctcccaccctgacaactctctgcccaccttgacctgcccaagtcgcgcggggacccgccctccccaccgcattcccatgcgtcccctggggggtcggggtggaggggccactgggaagggaacagaggccgggccgcccttcccccgctccgtagggggcgccccgggactccgcggccgccgtcgccaccgtcagacgcactgtccccgatccccgacccaccccgggcggcggggcgctcaaggcgcgcggggcggcgccctcgccttctcgcaacgctcttggggacccgccgggcgcagccccactccgcccacgagccaggcgcggaaaagttgccggcgccgctgccgccgaggcgccgatcgctcccggcctccctcctgggtccctcctgacttccacttacccgcggggggaggggagccgggcgcgcactccgggctccggccgccgccccgggccgggccggccgaggctcaggcgggcgggctgcgggcccgagaccggccgggggcggccgccggccgcgctccaccccactcactggcc

SEQ ID NO: 16660 - RNA, 63 nt, Homo sapiens
  source 1..63: mol_type = other RNA
gttcctgctgaactgagccagtgtgtaaaatgagaactgatatcagctcagtaggcaccggag

SEQ ID NO: 16661 - RNA, 2836 nt, Homo sapiens
  source 1..2836: mol_type = other RNA
gttcctgctgaactgagccagtgtgtaaaatgagaactgatatcagctcagtaggcaccggagggcgggtccaatcgacagcccggagaagcagcgcctcagctgggagctccgtgggcaccgtctgctggcgcaggagacgcgaaggcctggactcgttaaaataacatttcggccaccacctgggctgaggacctatccatctgctccttggtccgctcgaagcacctacgggcgagctgctgctgtctggcgtcctcactcaccatcagctccccgtagaggtacacacccatggcctgatcctcctgaaggaacctctccacacttttgtaggctttcgtgaacttgtgcttaacaatgagttcacaccaccgatggcgaacctctgcatcctgatcctggaggtggtatgtcctctggaggctttgcagagttcgggggctcagagtcttctgctccaagagatgctccagaagcaagaccagctggtctggaagaagcttttcaaacacctcttccttctccctgcgcttccgttttcggggtctccggttcactccaatccatttcgtgacctcggcgcgcacttgccgcgcaagcccgcactccgccccggcgcgacgctccctctgcagcggctttggtattccggaactctcaagccagtcttggtagatgttttcaacagacagctcaagccttttttcttctggaatgttctccagtagcatttgaaggaaatcctgggaaagaatcagctgtccatgaaatgtgtgcacaaattttcttaaaaatgaaaaataggtttcatctccaagtcttttggcaagaaaccgaagaaggaagtagccctttaaataatgcacctgcatgaagatcttctccggattaagtccatgcttgataacagatgctcccgagtcacttgtgtggccagttttgtctttactgggtcttaacacctgcatctcctcgggggagcattgcatctcgtcctggaggcgacgccagcgcagacaagccctcagctcctgctgctcccgggcctcatagggggccagctgctgtgctgtggcccaaaacacatcctccaagtgagtggcgaagccttcactcagccactcctccgtccagtctcgggccccgatggctaggccaaaccaggcatgggcaatttcatggcagaggcgggtcccacagagatggttccctcctgtcaagatgctctgagagaggaacatgatgtgtgggctggccatccccagacttggaaagttggcagggacgatgagaacatccagccgagagaacgggtgtgctcccagaacagaatgtgctgctgagaggcaaggagggatcagccgcagaagggtctcttggcaggcacccgtgaggcacacaggggcaaagacccgatgaggaatgatctcctgggtggtggcagaagcattctggaagcggcaggggtattccatgtgactgcaaacaccaacatgcctgaagttggcctcagaaggtgagaagggtctctctgttgccaaatcatttgatgaccatgtctccatcttcatttctgtccagcatcccactgcaattgtgaaggtggaggctggcattggcatagttacatagtaataccagcttgagcactcttcccaaagctgcgttggtttggcagaattttccccactcattaaaacaacaaaagatgcagctgctcgaactgtagcctgccatgttgacatggcaacgggtggctcctggcatggaaaaagggccctgttgtttatgggagatcccacagtataaacacatggcctgccactctggtctgaggtccatgtaaccgatcgcccttcaggtttagttttgtaccatatcctgatagcatgaggaaagtcagtagctgtctgagcccctgtcttccttatctgcaagctccaagtgtcagtgtcaaagaggagttccccacagccaggagcctggctgcagcgagcgtaatagtctaactgctccctccaacgatttgcaggcaaagtcacaagttcacgtacaatctgattcctgaactcctcagaaacaaccgtgagctcaggagaccttgtaaatttttccagacctggcacagcagcaacatccacctcctcgacttttaacacagataaatcacagcagtccaacactagcaaaaaatcctcactcccatgattccctgtgtcacagcagtactttgagctagaaatcccagaagcatgttcctggttgtcatggttaccatctttatcagaagtatctttttcacctttactacagattgcaaaatcattatattccatttcagatgagaaggtccttgcatttgtcacgggaatatggcagggttcaggcatcccaaatttgcaggctttgtttgattctgattggcaggcttcctcaatagagctattctgtttcttgaatctgtttccatcctcgaggaaaagcactatggtcccctcaatgacttgactttcaaaatccacatccaaatccagtacatagtgcttcacaagtatgtggctggtgttggccatgagaggcaggtcatctctggcagggtccagctgtatgtccatgatgtggtttattgtttgagggatttattaaaatctcagatggggtttcctatctgccttaatcttccagaatcataaatagctgcttatcaaagaaaacaactgatgtcacaaattatggttcctttcagtctcctgtctcagccgcgtcccacgggtcaccacttccgcagactcggggttactacgggctaccccggcacgcgccgggtgacgtc

SEQ ID NO: 16662 - RNA, 5705 nt, Homo sapiens
  source 1..5705: mol_type = other RNA
gttcctgctgaactgagccagtgtgtaaaatgagaactgatatcagctcagtaggcaccggagggcgggtccaatcgacagcccggagaagcagcgcctcagctgggagctccgtgggcaccgtctgctggcgcaggagacgcgaaggcctggactgcaaatacaagagagagttcaccgcgcccagaacaacaggagctcctccgaaagccccgccccgccccgctcacagccatgagctaccacatgatttcacacgacttaggtgatgcatttggttttagttttttgtaagaagaatttttgcaactttcaatacatttgacctttcagacagatgtccgattagtgcatgtttctgtggacagacttaaggactcagtacatggctagcattcccagcaggagacagtgcatccttggggtcaagtggtctctcatcctccaggatcgcgctccgcacccaagctgactgtgcagcagcggccggcccgtcagcaacggcctctgccccagcggctccaacttaactgtccccatctcaccttctcttcaggtgcagaacttagccactgtgaacaaagcggaaaccaatcactgttcaccaatcagctaagctctgcaccttgttagagaggtcatcgctgggcataaataaagggacggtgaccggtgagcatcttcctcagctggtggcttcttttgtttccaaagaagagctacgagatgcacctgttctccaatctgcagtgagcgcgaccacggtttctggaggagcagccaaggtcgtggttgcgtggtaatccctggcaatgtgattttaatcttaagtcacaaatcagcatgccaggaacccaagcagccagagcacctgagagcagcgccaccccgtgctgtctgcacacactgggcttccgcggaaggacgccggcgacactgccgccttcacgcctgttatgctagcaaacaggtggagtttctgtttgttgttcgtttagttggcatcctagaggtataatttcttgaatcaaagggactccagagatgaccataaaaatgccagtgcagctttggaactgaagaaaaatgcagggaccggccatgcgacacacacaattgctaaaggcagctgtccttgctattagtttactgcctctaacccttggggacaagatcccttctctccaggcagattctagctgccctgggaaggctttggggactctcaagtcaggaggtccccctgctggaaggggccctgggacaatcccggccactgttcctcacggggactggttggggggcaggcttgcaacccctggatgcatctggaggggtggggacaggatcgaagatgctggggagggggaaaagggagacttgtgaccaagatgactcctttgcctgcctgggcaaaaattccccataaagagtggcgaggggtgtgccctgtggtgctgctccaaaacctgcaccaaagggaatgatgaaaggactagctggccttgtagtttcacacactttaacacgtacgccacgaaataacaaaacgaaagagaaacaccatttacactgattactattatgaggccggcagtgaggtaagtgcacagtctgtgtgccgccagcccgtcctggaggggagccgcgtcaagtctgcagcaggcgtttcgctacgagacgctcagtcccgtttccctttcctggcacacatggttcctgactcttctggaagaatatgatcatgcttctgaaaaactttttatttcttttcattattagagttctttcagataaataagctacttaaacacgttacacagaaatggttttcataagcacaaaacattagaagaaaactcaatgttcaaaactgagtgaagaatatcaacaccaaatattcaatatccatgaaaaattatagagaagctataacacgaaaaatgcttcagatttgataaagtttttttaaagatacaaaattagacatcccctattaatatcatataaaacactgaagaaaaacggagcagacacagaaataatgatgattgttagagaaaaaaaatctcacagctatcctaacaaaaccttgtgtactaccgctaggttgctttaatagtgtagaaacccatactgagcaactaactgctaggaagtaaatctaacaggttaattccaggcacaattaacagaggaagtgatttaaataatctaggactccaatagaagccaggggagaaattccgctccaacacaacaaagcaaaaagtaggacctgccctcaagacacagggtcatggaggccatatgccacgtgtgctgtgtgcgccgcgggtgctgtgtggtgcgtgcactgtgtgtgccacatgtgctctgtgtggtgcgtgcggtgtgtgctgtgtgtgccgcaggtgctctgtgtggtgcacgcgctgtgtgtggtgtgtgtgctgcatgcagtgtgcgcgctacgtgtggtgcatgtgctgtgtgtgctctgtgttgtgcatgcgctgtgtgtggtgtgtgtgccgcgtgtactctgcgtggtgtgtgtgctgtgggtgctccaggtgctctgtgtggtgtgtgtgctgcgtgtgccgcgtgtgctctgtgtggtgcgtgcgctgtttggtgtgtatgctgcatgtgccgtgtgtgctctgcgtggtgcgtgcgctgtgtgtgctgtgtgtgccgcgtgtgctctgtgtggtgcgtgcgctgtgtggtgtgtgctgtgcgtgctctgtgtggtgcgtcctctggtgtgtgtgtgctgcatgcagtgtgtgtgctacgtgtggtgcatgtgctgtgtgtgctgcgtgtgcctggagagcctcctgccagccgatgaccaggcgtggacagcccaaggaacctccaattcacacatggctagaagaaaacatctgcttgcagaagctaggctttggagtcacacggccgcttaaactcctgtatcagccgtgaccctgaagactggaccagcgcttctgccaggcttcccattccatctctaaacctactcaagatgttcccccacaatttttgtttcaacagattataaaacctgaagtggccaaaatagtgccaaggagtgccgctgtgcctccaggtggacagcctctgcttcccggtgactgccacagccaggcaaggtgctccagggacccggggctcccataccagcccagcacccacttggccagttactctccaggccctgggccagggagccgactattgatgctgcgggtagtcttggctaactattcggcttactgatttagttggctcctaaaaggagtatctggttagaactaaatgacagaaaggaaagggagagaatcacctcgttaaaataacatttcggccaccacctgggctgaggacctatccatctgctccttggtccgctcgaagcacctacgggcgagctgctgctgtctggcgtcctcactcaccatcagctccccgtagaggtacacacccatggcctgatcctcctgaaggaacctctccacacttttgtaggctttcgtgaacttgtgcttaacaatgagttcacaccaccgatggcgaacctctgcatcctgatcctggaggtggtatgtcctctggaggctttgcagagttcgggggctcagagtcttctgctccaagagatgctccagaagcaagaccagctggtctggaagaagcttttcaaacacctcttccttctccctgcgcttccgttttcggggtctccggttcactccaatccatttcgtgacctcggcgcgcacttgccgcgcaagcccgcactccgccccggcgcgacgctccctctgcagcggctttggtattccggaactctcaagccagtcttggtagatgttttcaacagacagctcaagcctgggaaagaatcagctgtccatgaaatgtgtgcacaaattttcttaaaaatgaaaaataggtttcatctccaagtcttttggcaagaaaccgaagaaggaagtagccctttaaataatgcacctgcatgaagatcttctccggattaagtccatgcttgataacagatgctcccgagtcacttgtgtggccagttttgtctttactgggtctggccatccccagacttggaaagttggcagggacgatgagaacatccagccgagagaacgggtgtgctcccagaacagaatgtgctgctgagaggcaaggagggatcagccgcagaagggtctcttggcaggcacccgtgaggcacacaggggcaaagacccgatgaggaatgatctcctgggtggtggcagaagcattctggaagcggcaggggtattccatgtgactgcaaacaccaacatgcctgaagttggcctcagaaggtgagaagggtctctctgttgccaaatcatttgatgaccatgtctccatcttcatttctgtccagcatcccactgcaattgtgaaggtggaggctggcattggcatagttacatagtaataccagcttgagcactcttcccaaagctgcgttggtttggcagaattttccccactcattaaaacaacaaaagatgcagctgctcgaactgtagcctgccatgttgacatggcaacgggtggctcctggcatggaaaaagggccctgttgtttatgggagatcccacagtataaacacatggcctgccactctggtctgaggtccatgtaaccgatcgcccttcaggtttagttttgtaccatatcctgatagcatgaggaaagtcagtagctgtctgagcccctgtcttccttatctgcaagctccaagtgtcagtgtcaaagaggagttccccacagccaggagcctggctgcagcgagcgtaatagtctaactgctccctccaacgatttgcaggcaaagtcacaagttcacgtacaatctgattcctgaactcctcagaaacaaccgtgagctcaggagaccttgtaaatttttccagacctggcacagcagcaacatccacctcctcgacttttaacacagataaatcacagcagtccaacactagcaaaaaatcctcactcccatgattccctgtgtcacagcagtactttgagctagaaatcccagaagcatgttcctggttgtcatggttaccatctttatcagaagtatctttttcacctttactacagattgcaaaatcattatattccatttcagatgagaaggtccttgcatttgtcacgggaatatggcagggttcaggcatcccaaatttgcaggctttgtttgattctgattggcaggcttcctcaatagagctattctgtttcttgaatctgtttccatcctcgaggaaaagcactatggtcccctcaatgacttgactttcaaaatccacatccaaatccagtacatagtgcttcacaagtatgtggctggtgttggccatgagaggcaggtcatctctggcagggtccagctgtatgtccatgatgtggtttattgtttgagggatttattaaaatctcagatggggtttcctatctgccttaatcttccagaatcataaatagctgcttatcaaagaaaacaactgatgtcacaaattatggttcctttcagtctcctgtctcagccgcgtcccacgggtcaccacttccgcagactcggggttactacgggctaccccggcacgcgccgggtgacgtc

SEQ ID NO: 16663 - RNA, 5582 nt, Homo sapiens
  source 1..5582: mol_type = other RNA
gttcctgctgaactgagccagtgtgtaaaatgagaactgatatcagctcagtaggcaccggagggcgggtccaatcgacagcccggagaagcagcgcctcagctgggagctccgtgggcaccgtctgctggcgcaggagacgcgaaggcctggactgcaaatacaagagagagttcaccgcgcccagaacaacaggagctcctccgaaagccccgccccgccccgctcacagccatgagctaccacatgatttcacacgacttaggtgatgcatttggttttagttttttgtaagaagaatttttgcaactttcaatacatttgacctttcagacagatgtccgattagtgcatgtttctgtggacagacttaaggactcagtacatggctagcattcccagcaggagacagtgcatccttggggtcaagtggtctctcatcctccaggatcgcgctccgcacccaagctgactgtgcagcagcggccggcccgtcagcaacggcctctgccccagcggctccaacttaactgtccccatctcaccttctcttcaggtgcagaacttagccactgtgaacaaagcggaaaccaatcactgttcaccaatcagctaagctctgcaccttgttagagaggtcatcgctgggcataaataaagggacggtgaccggtgagcatcttcctcagctggtggcttcttttgtttccaaagaagagctacgagatgcacctgttctccaatctgcagtgagcgcgaccacggtttctggaggagcagccaaggtcgtggttgcgtggtaatccctggcaatgtgattttaatcttaagtcacaaatcagcatgccaggaacccaagcagccagagcacctgagagcagcgccaccccgtgctgtctgcacacactgggcttccgcggaaggacgccggcgacactgccgccttcacgcctgttatgctagcaaacaggtggagtttctgtttgttgttcgtttagttggcatcctagaggtataatttcttgaatcaaagggactccagagatgaccataaaaatgccagtgcagctttggaactgaagaaaaatgcagggaccggccatgcgacacacacaattgctaaaggcagctgtccttgctattagtttactgcctctaacccttggggacaagatcccttctctccaggcagattctagctgccctgggaaggctttggggactctcaagtcaggaggtccccctgctggaaggggccctgggacaatcccggccactgttcctcacggggactggttggggggcaggcttgcaacccctggatgcatctggaggggtggggacaggatcgaagatgctggggagggggaaaagggagacttgtgaccaagatgactcctttgcctgcctgggcaaaaattccccataaagagtggcgaggggtgtgccctgtggtgctgctccaaaacctgcaccaaagggaatgatgaaaggactagctggccttgtagtttcacacactttaacacgtacgccacgaaataacaaaacgaaagagaaacaccatttacactgattactattatgaggccggcagtgaggtaagtgcacagtctgtgtgccgccagcccgtcctggaggggagccgcgtcaagtctgcagcaggcgtttcgctacgagacgctcagtcccgtttccctttcctggcacacatggttcctgactcttctggaagaatatgatcatgcttctgaaaaactttttatttcttttcattattagagttctttcagataaataagctacttaaacacgttacacagaaatggttttcataagcacaaaacattagaagaaaactcaatgttcaaaactgagtgaagaatatcaacaccaaatattcaatatccatgaaaaattatagagaagctataacacgaaaaatgcttcagatttgataaagtttttttaaagatacaaaattagacatcccctattaatatcatataaaacactgaagaaaaacggagcagacacagaaataatgatgattgttagagaaaaaaaatctcacagctatcctaacaaaaccttgtgtactaccgctaggttgctttaatagtgtagaaacccatactgagcaactaactgctaggaagtaaatctaacaggttaattccaggcacaattaacagaggaagtgatttaaataatctaggactccaatagaagccaggggagaaattccgctccaacacaacaaagcaaaaagtaggacctgccctcaagacacagggtcatggaggccatatgccacgtgtgctgtgtgcgccgcgggtgctgtgtggtgcgtgcactgtgtgtgccacatgtgctctgtgtggtgcgtgcggtgtgtgctgtgtgtgccgcaggtgctctgtgtggtgcacgcgctgtgtgtggtgtgtgtgctgcatgcagtgtgcgcgctacgtgtggtgcatgtgctgtgtgtgctctgtgttgtgcatgcgctgtgtgtggtgtgtgtgccgcgtgtactctgcgtggtgtgtgtgctgtgggtgctccaggtgctctgtgtggtgtgtgtgctgcgtgtgccgcgtgtgctctgtgtggtgcgtgcgctgtttggtgtgtatgctgcatgtgccgtgtgtgctctgcgtggtgcgtgcgctgtgtgtgctgtgtgtgccgcgtgtgctctgtgtggtgcgtgcgctgtgtggtgtgtgctgtgcgtgctctgtgtggtgcgtcctctggtgtgtgtgtgctgcatgcagtgtgtgtgctacgtgtggtgcatgtgctgtgtgtgctgcgtgtgcctggagagcctcctgccagccgatgaccaggcgtggacagcccaaggaacctccaattcacacatggctagaagaaaacatctgcttgcagaagctaggctttggagtcacacggccgcttaaactcctgtatcagccgtgaccctgaagactggaccagcgcttctgccaggcttcccattccatctctaaacctactcaagatgttcccccacaatttttgtttcaacagattataaaacctgaagtggccaaaatagtgccaaggagtgccgctgtgcctccaggtggacagcctctgcttcccggtgactgccacagccaggcaaggtgctccagggacccggggctcccataccagcccagcacccacttggccagttactctccaggccctgggccagggagccgactattgatgctgcgggtagtcttggctaactattcggcttactgatttagttggctcctaaaaggagtatctggttagaactaaatgacagaaaggaaagggagagaatcacctcgttaaaataacatttcggccaccacctgggctgaggacctatccatctgctccttggtccgctcgaagcacctacgggcgagctgctgctgtctggcgtcctcactcaccatcagctccccgtagaggtacacacccatggcctgatcctcctgaaggaacctctccacacttttgtaggctttcgtgaacttgtgcttaacaatgagttcacaccaccgatggcgaacctctgcatcctgatcctggaggtggtatgtcctctggaggctttgcagagttcgggggctcagagtcttctgctccaagagatgctccagaagcaagaccagctggtctggaagaagcttttcaaacacctcttccttctccctgcgcttccgttttcggggtctccggttcactccaatccatttcgtgacctcggcgcgcacttgccgcgcaagcccgcactccgccccggcgcgacgctccctctgcagcggctttggtattccggaactctcaagccagtcttggtagatgttttcaacagacagctcaagccttttttcttctggaatgttctccagtagcatttgaaggaaatcctgggaaagaatcagctgtccatgaaatgtgtgcacaaattttcttaaaaatgaaaaataggtttcatctccaagtcttttggcaagaaaccgaagaaggaagtagccctttaaataatgcacctgcatgaagatcttctccggattaagtccatgcttgataacagatgctcccgagtcacttgtgtggccagttttgtctttactgggtctggccatccccagacttggaaagttggcagggacgatgagaacatccagccgagagaacgggtgtgctcccagaacagaatgtgctgctgagaggcaaggagggatcagccgcagaagggtctcttggcaggcacccgtgaggcacacaggggcaaagacccgatgaggaatgatctcctgggtggtggcagaagcattctggaagcggcaggggtattccatgtgactgcaaacaccaacatgcctgaagttggcctcagaaggtgagaagggtctctctgttgccaaatcatttgatgaccatgtctccatcttcatttctgtccagcatcccactgcaattgtgaaggtggaggctggcattggcatagttacatagtaataccagcttgagcactctgccactctggtctgaggtccatgtaaccgatcgcccttcaggtttagttttgtaccatatcctgatagcatgaggaaagtcagtagctgtctgagcccctgtcttccttatctgcaagctccaagtgtcagtgtcaaagaggagttccccacagccaggagcctggctgcagcgagcgtaatagtctaactgctccctccaacgatttgcaggcaaagtcacaagttcacgtacaatctgattcctgaactcctcagaaacaaccgtgagctcaggagaccttgtaaatttttccagacctggcacagcagcaacatccacctcctcgacttttaacacagataaatcacagcagtccaacactagcaaaaaatcctcactcccatgattccctgtgtcacagcagtactttgagctagaaatcccagaagcatgttcctggttgtcatggttaccatctttatcagaagtatctttttcacctttactacagattgcaaaatcattatattccatttcagatgagaaggtccttgcatttgtcacgggaatatggcagggttcaggcatcccaaatttgcaggctttgtttgattctgattggcaggcttcctcaatagagctattctgtttcttgaatctgtttccatcctcgaggaaaagcactatggtcccctcaatgacttgactttcaaaatccacatccaaatccagtacatagtgcttcacaagtatgtggctggtgttggccatgagaggcaggtcatctctggcagggtccagctgtatgtccatgatgtggtttattgtttgagggatttattaaaatctcagatggggtttcctatctgccttaatcttccagaatcataaatagctgcttatcaaagaaaacaactgatgtcacaaattatggttcctttcagtctcctgtctcagccgcgtcccacgggtcaccacttccgcagactcggggttactacgggctaccccggcacgcgccgggtgacgtc

SEQ ID NO: 16664 - RNA, 5749 nt, Homo sapiens
  source 1..5749: mol_type = other RNA
gttcctgctgaactgagccagtgtgtaaaatgagaactgatatcagctcagtaggcaccggagggcgggtccaatcgacagcccggagaagcagcgcctcagctgggagctccgtgggcaccgtctgctggcgcaggagacgcgaaggcctggactgcaaatacaagagagagttcaccgcgcccagaacaacaggagctcctccgaaagccccgccccgccccgctcacagccatgagctaccacatgatttcacacgacttaggtgatgcatttggttttagttttttgtaagaagaatttttgcaactttcaatacatttgacctttcagacagatgtccgattagtgcatgtttctgtggacagacttaaggactcagtacatggctagcattcccagcaggagacagtgcatccttggggtcaagtggtctctcatcctccaggatcgcgctccgcacccaagctgactgtgcagcagcggccggcccgtcagcaacggcctctgccccagcggctccaacttaactgtccccatctcaccttctcttcaggtgcagaacttagccactgtgaacaaagcggaaaccaatcactgttcaccaatcagctaagctctgcaccttgttagagaggtcatcgctgggcataaataaagggacggtgaccggtgagcatcttcctcagctggtggcttcttttgtttccaaagaagagctacgagatgcacctgttctccaatctgcagtgagcgcgaccacggtttctggaggagcagccaaggtcgtggttgcgtggtaatccctggcaatgtgattttaatcttaagtcacaaatcagcatgccaggaacccaagcagccagagcacctgagagcagcgccaccccgtgctgtctgcacacactgggcttccgcggaaggacgccggcgacactgccgccttcacgcctgttatgctagcaaacaggtggagtttctgtttgttgttcgtttagttggcatcctagaggtataatttcttgaatcaaagggactccagagatgaccataaaaatgccagtgcagctttggaactgaagaaaaatgcagggaccggccatgcgacacacacaattgctaaaggcagctgtccttgctattagtttactgcctctaacccttggggacaagatcccttctctccaggcagattctagctgccctgggaaggctttggggactctcaagtcaggaggtccccctgctggaaggggccctgggacaatcccggccactgttcctcacggggactggttggggggcaggcttgcaacccctggatgcatctggaggggtggggacaggatcgaagatgctggggagggggaaaagggagacttgtgaccaagatgactcctttgcctgcctgggcaaaaattccccataaagagtggcgaggggtgtgccctgtggtgctgctccaaaacctgcaccaaagggaatgatgaaaggactagctggccttgtagtttcacacactttaacacgtacgccacgaaataacaaaacgaaagagaaacaccatttacactgattactattatgaggccggcagtgaggtaagtgcacagtctgtgtgccgccagcccgtcctggaggggagccgcgtcaagtctgcagcaggcgtttcgctacgagacgctcagtcccgtttccctttcctggcacacatggttcctgactcttctggaagaatatgatcatgcttctgaaaaactttttatttcttttcattattagagttctttcagataaataagctacttaaacacgttacacagaaatggttttcataagcacaaaacattagaagaaaactcaatgttcaaaactgagtgaagaatatcaacaccaaatattcaatatccatgaaaaattatagagaagctataacacgaaaaatgcttcagatttgataaagtttttttaaagatacaaaattagacatcccctattaatatcatataaaacactgaagaaaaacggagcagacacagaaataatgatgattgttagagaaaaaaaatctcacagctatcctaacaaaaccttgtgtactaccgctaggttgctttaatagtgtagaaacccatactgagcaactaactgctaggaagtaaatctaacaggttaattccaggcacaattaacagaggaagtgatttaaataatctaggactccaatagaagccaggggagaaattccgctccaacacaacaaagcaaaaagtaggacctgccctcaagacacagggtcatggaggccatatgccacgtgtgctgtgtgcgccgcgggtgctgtgtggtgcgtgcactgtgtgtgccacatgtgctctgtgtggtgcgtgcggtgtgtgctgtgtgtgccgcaggtgctctgtgtggtgcacgcgctgtgtgtggtgtgtgtgctgcatgcagtgtgcgcgctacgtgtggtgcatgtgctgtgtgtgctctgtgttgtgcatgcgctgtgtgtggtgtgtgtgccgcgtgtactctgcgtggtgtgtgtgctgtgggtgctccaggtgctctgtgtggtgtgtgtgctgcgtgtgccgcgtgtgctctgtgtggtgcgtgcgctgtttggtgtgtatgctgcatgtgccgtgtgtgctctgcgtggtgcgtgcgctgtgtgtgctgtgtgtgccgcgtgtgctctgtgtggtgcgtgcgctgtgtggtgtgtgctgtgcgtgctctgtgtggtgcgtcctctggtgtgtgtgtgctgcatgcagtgtgtgtgctacgtgtggtgcatgtgctgtgtgtgctgcgtgtgcctggagagcctcctgccagccgatgaccaggcgtggacagcccaaggaacctccaattcacacatggctagaagaaaacatctgcttgcagaagctaggctttggagtcacacggccgcttaaactcctgtatcagccgtgaccctgaagactggaccagcgcttctgccaggcttcccattccatctctaaacctactcaagatgttcccccacaatttttgtttcaacagattataaaacctgaagtggccaaaatagtgccaaggagtgccgctgtgcctccaggtggacagcctctgcttcccggtgactgccacagccaggcaaggtgctccagggacccggggctcccataccagcccagcacccacttggccagttactctccaggccctgggccagggagccgactattgatgctgcgggtagtcttggctaactattcggcttactgatttagttggctcctaaaaggagtatctggttagaactaaatgacagaaaggaaagggagagaatcacctcgttaaaataacatttcggccaccacctgggctgaggacctatccatctgctccttggtccgctcgaagcacctacgggcgagctgctgctgtctggcgtcctcactcaccatcagctccccgtagaggtacacacccatggcctgatcctcctgaaggaacctctccacacttttgtaggctttcgtgaacttgtgcttaacaatgagttcacaccaccgatggcgaacctctgcatcctgatcctggaggtggtatgtcctctggaggctttgcagagttcgggggctcagagtcttctgctccaagagatgctccagaagcaagaccagctggtctggaagaagcttttcaaacacctcttccttctccctgcgcttccgttttcggggtctccggttcactccaatccatttcgtgacctcggcgcgcacttgccgcgcaagcccgcactccgccccggcgcgacgctccctctgcagcggctttggtattccggaactctcaagccagtcttggtagatgttttcaacagacagctcaagccttttttcttctggaatgttctccagtagcatttgaaggaaatcctgggaaagaatcagctgtccatgaaatgtgtgcacaaattttcttaaaaatgaaaaataggtttcatctccaagtcttttggcaagaaaccgaagaaggaagtagccctttaaataatgcacctgcatgaagatcttctccggattaagtccatgcttgataacagatgctcccgagtcacttgtgtggccagttttgtctttactgggtctggccatccccagacttggaaagttggcagggacgatgagaacatccagccgagagaacgggtgtgctcccagaacagaatgtgctgctgagaggcaaggagggatcagccgcagaagggtctcttggcaggcacccgtgaggcacacaggggcaaagacccgatgaggaatgatctcctgggtggtggcagaagcattctggaagcggcaggggtattccatgtgactgcaaacaccaacatgcctgaagttggcctcagaaggtgagaagggtctctctgttgccaaatcatttgatgaccatgtctccatcttcatttctgtccagcatcccactgcaattgtgaaggtggaggctggcattggcatagttacatagtaataccagcttgagcactcttcccaaagctgcgttggtttggcagaattttccccactcattaaaacaacaaaagatgcagctgctcgaactgtagcctgccatgttgacatggcaacgggtggctcctggcatggaaaaagggccctgttgtttatgggagatcccacagtataaacacatggcctgccactctggtctgaggtccatgtaaccgatcgcccttcaggtttagttttgtaccatatcctgatagcatgaggaaagtcagtagctgtctgagcccctgtcttccttatctgcaagctccaagtgtcagtgtcaaagaggagttccccacagccaggagcctggctgcagcgagcgtaatagtctaactgctccctccaacgatttgcaggcaaagtcacaagttcacgtacaatctgattcctgaactcctcagaaacaaccgtgagctcaggagaccttgtaaatttttccagacctggcacagcagcaacatccacctcctcgacttttaacacagataaatcacagcagtccaacactagcaaaaaatcctcactcccatgattccctgtgtcacagcagtactttgagctagaaatcccagaagcatgttcctggttgtcatggttaccatctttatcagaagtatctttttcacctttactacagattgcaaaatcattatattccatttcagatgagaaggtccttgcatttgtcacgggaatatggcagggttcaggcatcccaaatttgcaggctttgtttgattctgattggcaggcttcctcaatagagctattctgtttcttgaatctgtttccatcctcgaggaaaagcactatggtcccctcaatgacttgactttcaaaatccacatccaaatccagtacatagtgcttcacaagtatgtggctggtgttggccatgagaggcaggtcatctctggcagggtccagctgtatgtccatgatgtggtttattgtttgagggatttattaaaatctcagatggggtttcctatctgccttaatcttccagaatcataaatagctgcttatcaaagaaaacaactgatgtcacaaattatggttcctttcagtctcctgtctcagccgcgtcccacgggtcaccacttccgcagactcggggttactacgggctaccccggcacgcgccgggtgacgtc

SEQ ID NO: 16665 - RNA, 6046 nt, Homo sapiens
  source 1..6046: mol_type = other RNA
gttcctgctgaactgagccagtgtgtaaaatgagaactgatatcagctcagtaggcaccggagggcgggtccaatcgacagcccggagaagcagcgcctcagctgggagctccgtgggcaccgtctgctggcgcaggagacgcgaaggcctggactgcaaatacaagagagagttcaccgcgcccagaacaacaggagctcctccgaaagccccgccccgccccgctcacagccatgagctaccacatgatttcacacgacttaggtgatgcatttggttttagttttttgtaagaagaatttttgcaactttcaatacatttgacctttcagacagatgtccgattagtgcatgtttctgtggacagacttaaggactcagtacatggctagcattcccagcaggagacagtgcatccttggggtcaagtggtctctcatcctccaggatcgcgctccgcacccaagctgactgtgcagcagcggccggcccgtcagcaacggcctctgccccagcggctccaacttaactgtccccatctcaccttctcttcaggtgcagaacttagccactgtgaacaaagcggaaaccaatcactgttcaccaatcagctaagctctgcaccttgttagagaggtcatcgctgggcataaataaagggacggtgaccggtgagcatcttcctcagctggtggcttcttttgtttccaaagaagagctacgagatgcacctgttctccaatctgcagtgagcgcgaccacggtttctggaggagcagccaaggtcgtggttgcgtggtaatccctggcaatgtgattttaatcttaagtcacaaatcagcatgccaggaacccaagcagccagagcacctgagagcagcgccaccccgtgctgtctgcacacactgggcttccgcggaaggacgccggcgacactgccgccttcacgcctgttatgctagcaaacaggtggagtttctgtttgttgttcgtttagttggcatcctagaggtataatttcttgaatcaaagggactccagagatgaccataaaaatgccagtgcagctttggaactgaagaaaaatgcagggaccggccatgcgacacacacaattgctaaaggcagctgtccttgctattagtttactgcctctaacccttggggacaagatcccttctctccaggcagattctagctgccctgggaaggctttggggactctcaagtcaggaggtccccctgctggaaggggccctgggacaatcccggccactgttcctcacggggactggttggggggcaggcttgcaacccctggatgcatctggaggggtggggacaggatcgaagatgctggggagggggaaaagggagacttgtgaccaagatgactcctttgcctgcctgggcaaaaattccccataaagagtggcgaggggtgtgccctgtggtgctgctccaaaacctgcaccaaagggaatgatgaaaggactagctggccttgtagtttcacacactttaacacgtacgccacgaaataacaaaacgaaagagaaacaccatttacactgattactattatgaggccggcagtgaggtaagtgcacagtctgtgtgccgccagcccgtcctggaggggagccgcgtcaagtctgcagcaggcgtttcgctacgagacgctcagtcccgtttccctttcctggcacacatggttcctgactcttctggaagaatatgatcatgcttctgaaaaactttttatttcttttcattattagagttctttcagataaataagctacttaaacacgttacacagaaatggttttcataagcacaaaacattagaagaaaactcaatgttcaaaactgagtgaagaatatcaacaccaaatattcaatatccatgaaaaattatagagaagctataacacgaaaaatgcttcagatttgataaagtttttttaaagatacaaaattagacatcccctattaatatcatataaaacactgaagaaaaacggagcagacacagaaataatgatgattgttagagaaaaaaaatctcacagctatcctaacaaaaccttgtgtactaccgctaggttgctttaatagtgtagaaacccatactgagcaactaactgctaggaagtaaatctaacaggttaattccaggcacaattaacagaggaagtgatttaaataatctaggactccaatagaagccaggggagaaattccgctccaacacaacaaagcaaaaagtaggacctgccctcaagacacagggtcatggaggccatatgccacgtgtgctgtgtgcgccgcgggtgctgtgtggtgcgtgcactgtgtgtgccacatgtgctctgtgtggtgcgtgcggtgtgtgctgtgtgtgccgcaggtgctctgtgtggtgcacgcgctgtgtgtggtgtgtgtgctgcatgcagtgtgcgcgctacgtgtggtgcatgtgctgtgtgtgctctgtgttgtgcatgcgctgtgtgtggtgtgtgtgccgcgtgtactctgcgtggtgtgtgtgctgtgggtgctccaggtgctctgtgtggtgtgtgtgctgcgtgtgccgcgtgtgctctgtgtggtgcgtgcgctgtttggtgtgtatgctgcatgtgccgtgtgtgctctgcgtggtgcgtgcgctgtgtgtgctgtgtgtgccgcgtgtgctctgtgtggtgcgtgcgctgtgtggtgtgtgctgtgcgtgctctgtgtggtgcgtcctctggtgtgtgtgtgctgcatgcagtgtgtgtgctacgtgtggtgcatgtgctgtgtgtgctgcgtgtgcctggagagcctcctgccagccgatgaccaggcgtggacagcccaaggaacctccaattcacacatggctagaagaaaacatctgcttgcagaagctaggctttggagtcacacggccgcttaaactcctgtatcagccgtgaccctgaagactggaccagcgcttctgccaggcttcccattccatctctaaacctactcaagatgttcccccacaatttttgtttcaacagattataaaacctgaagtggccaaaatagtgccaaggagtgccgctgtgcctccaggtggacagcctctgcttcccggtgactgccacagccaggcaaggtgctccagggacccggggctcccataccagcccagcacccacttggccagttactctccaggccctgggccagggagccgactattgatgctgcgggtagtcttggctaactattcggcttactgatttagttggctcctaaaaggagtatctggttagaactaaatgacagaaaggaaagggagagaatcacctcgttaaaataacatttcggccaccacctgggctgaggacctatccatctgctccttggtccgctcgaagcacctacgggcgagctgctgctgtctggcgtcctcactcaccatcagctccccgtagaggtacacacccatggcctgatcctcctgaaggaacctctccacacttttgtaggctttcgtgaacttgtgcttaacaatgagttcacaccaccgatggcgaacctctgcatcctgatcctggaggtggtatgtcctctggaggctttgcagagttcgggggctcagagtcttctgctccaagagatgctccagaagcaagaccagctggtctggaagaagcttttcaaacacctcttccttctccctgcgcttccgttttcggggtctccggttcactccaatccatttcgtgacctcggcgcgcacttgccgcgcaagcccgcactccgccccggcgcgacgctccctctgcagcggctttggtattccggaactctcaagccagtcttggtagatgttttcaacagacagctcaagccttttttcttctggaatgttctccagtagcatttgaaggaaatcctgggaaagaatcagctgtccatgaaatgtgtgcacaaattttcttaaaaatgaaaaataggtttcatctccaagtcttttggcaagaaaccgaagaaggaagtagccctttaaataatgcacctgcatgaagatcttctccggattaagtccatgcttgataacagatgctcccgagtcacttgtgtggccagttttgtctttactgggtcttaacacctgcatctcctcgggggagcattgcatctcgtcctggaggcgacgccagcgcagacaagccctcagctcctgctgctcccgggcctcatagggggccagctgctgtgctgtggcccaaaacacatcctccaagtgagtggcgaagccttcactcagccactcctccgtccagtctcgggccccgatggctaggccaaaccaggcatgggcaatttcatggcagaggcgggtcccacagagatggttccctcctgtcaagatgctctgagagaggaacatgatgtgtgggctggccatccccagacttggaaagttggcagggacgatgagaacatccagccgagagaacgggtgtgctcccagaacagaatgtgctgctgagaggcaaggagggatcagccgcagaagggtctcttggcaggcacccgtgaggcacacaggggcaaagacccgatgaggaatgatctcctgggtggtggcagaagcattctggaagcggcaggggtattccatgtgactgcaaacaccaacatgcctgaagttggcctcagaaggtgagaagggtctctctgttgccaaatcatttgatgaccatgtctccatcttcatttctgtccagcatcccactgcaattgtgaaggtggaggctggcattggcatagttacatagtaataccagcttgagcactcttcccaaagctgcgttggtttggcagaattttccccactcattaaaacaacaaaagatgcagctgctcgaactgtagcctgccatgttgacatggcaacgggtggctcctggcatggaaaaagggccctgttgtttatgggagatcccacagtataaacacatggcctgccactctggtctgaggtccatgtaaccgatcgcccttcaggtttagttttgtaccatatcctgatagcatgaggaaagtcagtagctgtctgagcccctgtcttccttatctgcaagctccaagtgtcagtgtcaaagaggagttccccacagccaggagcctggctgcagcgagcgtaatagtctaactgctccctccaacgatttgcaggcaaagtcacaagttcacgtacaatctgattcctgaactcctcagaaacaaccgtgagctcaggagaccttgtaaatttttccagacctggcacagcagcaacatccacctcctcgacttttaacacagataaatcacagcagtccaacactagcaaaaaatcctcactcccatgattccctgtgtcacagcagtactttgagctagaaatcccagaagcatgttcctggttgtcatggttaccatctttatcagaagtatctttttcacctttactacagattgcaaaatcattatattccatttcagatgagaaggtccttgcatttgtcacgggaatatggcagggttcaggcatcccaaatttgcaggctttgtttgattctgattggcaggcttcctcaatagagctattctgtttcttgaatctgtttccatcctcgaggaaaagcactatggtcccctcaatgacttgactttcaaaatccacatccaaatccagtacatagtgcttcacaagtatgtggctggtgttggccatgagaggcaggtcatctctggcagggtccagctgtatgtccatgatgtggtttattgtttgagggatttattaaaatctcagatggggtttcctatctgccttaatcttccagaatcataaatagctgcttatcaaagaaaacaactgatgtcacaaattatggttcctttcagtctcctgtctcagccgcgtcccacgggtcaccacttccgcagactcggggttactacgggctaccccggcacgcgccgggtgacgtc

SEQ ID NO: 16666 - RNA, 647 nt, Homo sapiens
  source 1..647: mol_type = other RNA
gtttgcacgggtgggccttgtctgatcagttgaagggcttagaatgttcatcatacttctccaagactcggtttccccatctggaaagtcaccatgctgggagacactggtttctaggtctgttgtgaacacaagaggagatgaggcagctggagcaggcatcattgtgttacagttgcttacagtatcccttatagtacctgtacatgctgtacaggtgtgtaggttaggaacaataggatctgccacacagcctgggcctacaggagactatgccatctaggtttgagtcagtatactctacgatgagcaaacaatgacagaatcacctaatgacacatttctccctccctcttcctattgttacgcaatatatgattgtatttcctgacagaactgtgctacaaagaccctcccatggtgattgtgaatcttccaaattttccctgtaatcctttcagttcttaaaaatatttttgaaattatgttattatttgtatttaatgttcacattcctgtgtctccttgatcaattttccattggccctttttaaaaattggaattattctttttgttgccttatgttattttcgcaagcatatgccttgagtataattctctctctttctctgtgtctccttttaaa

SEQ ID NO: 16667 - RNA, 1478 nt, Homo sapiens
  source 1..1478: mol_type = other RNA
gttttaccacctccaggagactggagatttgggcatgtgaggctggcctccaggtgacaggaccgcagggcaggctggccaggagctgggagccggcgcagcctcacttgagattgtgctggctctcgcggtgccgccgcaggtccaccttgcgctggaagcctttggtgcacagctcacagctgaagggcttgaagcctgtgtgcttgcggctgtgggtgatgaggttggagctctggctgaaggcctttccgcacacctggcacttgtgcggcttctcacctgtgtggatgtaggtgtgcttcttcatgtcggacttctggtggaaacgcttgccgcagaactggcaggggtagggccgcgtgtctgagtggatgagcaggtgggtggacagcgtggacgagcgcttgaaggccttgccgcacatgcggcactcgaagctgcgctcctgccggaggaaatgaggccccggggggtcaggtgcaggctcaggactggacccggccgggatcccctgggagtggacgtgcgtgtgctgctccaggctcacagcgtggccgaaggttttgccgcagatgtcacaggcgaagggccgggtcccactatgggagcgtcgcacatgcacttcgagcccgtgaggggtggagaagaccttgttgcacttcacacagtggtacgcatccatgcctggggagtagcggaggctgaagtccaaggcgggctcagtgctgggcacaagaggactgccgtacaggctgacggagtgctccaggaaggctgactgcatggtggagggggcctgccggtagctgtggccataggttgtggccaaggtgtcccaggagaagctaggcttgtagaatgggggtgagtcggacagtggagagtccccatcctggggtcgggacagcacaatggggccctctggtgccggggccatcctggccaagttctggtcctgctccagctccggctctcgtttgaggttggtccagtccaggcactggtttgggaatagagtgctaaggacagggctgttgcttggagcctggtctctgggcaccggggtaagggcaggaggccagagcggttcatcttcctgcacacggggctggtggtaggtgtgagccttcttgctcttcaccaggaaggagcgtggcattttcagtgtgcaccccacacccacggcgattctgcagacctcctcttcacaagtcctgttttagagtgagcatgtctcctcagatgcctcaacacttaaacttggttttttttctccaaaaataggtggaaagggctaacaacagccacagggaaaggcgagctgaaacagtacctctccatggtcggtcctattgttcctggagcctgggcagtgtgtgggagagggcagccctgtcatctccccttagtaggctctggaggggagagcgcctgactctcaaagtgtcctgggaatttggctgggcgcagtggct

SEQ ID NO: 16668 - RNA, 1330 nt, Homo sapiens
  source 1..1330: mol_type = other RNA
gttttaccacctccaggagactggagatttgggcatgtgaggctggcctccaggtgacaggaccgcagggcaggctggccaggagctgggagccggcgcagcctcacttgagattgtgctggctctcgcggtgccgccgcaggtccaccttgcgctggaagcctttggtgcacagctcacagctgaagggcttgaagcctgtgtgcttgcggctgtgggtgatgaggttggagctctggctgaaggcctttccgcacacctggcacttgtgcggcttctcacctgtgtggatgtaggtgtgcttcttcatgtcggacttctggtggaaacgcttgccgcagaactggcaggggtagggccgcgtgtctgagtggatgagcaggtgggtggacagcgtggacgagcgcttgaaggccttgccgcacatgcggcactcgaagctgcgctcctgccggaggaaatgaggccccggggggtcaggtgcaggctcaggactggacccggccgggatcccctgggagtggacgtgcgtgtgctgctccaggctcacagcgtggccgaaggttttgccgcagatgtcacaggcgaagggccgggtcccactatgggagcgtcgcacatgcacttcgagcccgtgaggggtggagaagaccttgttgcacttcacacagtggtacgcatccatgcctggggagtagcggaggctgaagtccaaggcgggctcagtgctgggcacaagaggactgccgtacaggctgacggagtgctccaggaaggctgactgcatggtggagggggcctgccggtagctgtggccataggttgtggccaaggtgtcccaggagaagctaggcttgtagaatgggggtgagtcggacagtggagagtccccatcctggggtcgggacagcacaatggggccctctggtgccggggccatcctggccaagttctggtcctgctccagctccggctctcgtttgaggttggtccagtccaggcactggtttgggaatagagtgctaaggacagggctgttgcttggagcctggtctctgggcaccggggtaagggcaggaggccagagcggttcatcttcctgcacacggggctggtggtaggtgtgagccttcttgctcttcaccaggaaggagcgtggcattttcagtgtgcaccccacacctgtccggagctgtccctcgcctgggttctgccggagcttcccgaggtgggaactgcaaagcctctctcgggactggcctccactctgtcaactgtgtgactctttgcacaaatagatacttctcctttttgctctgtctctctgtgt

SEQ ID NO: 16669 - RNA, 1878 nt, Homo sapiens
  source 1..1878: mol_type = other RNA
gttttaccacctccaggagactggagatttgggcatgtgaggctggcctccaggtgacaggaccgcagggcaggctggccaggagctgggagccggcgcagcctcacttgagattgtgctggctctcgcggtgccgccgcaggtccaccttgcgctggaagcctttggtgcacagctcacagctgaagggcttgaagcctgtgtgcttgcggctgtgggtgatgaggttggagctctggctgaaggcctttccgcacacctggcacttgtgcggcttctcacctgtgtggatgtaggtgtgcttcttcatgtcggacttctggtggaaacgcttgccgcagaactggcaggggtagggccgcgtgtctgagtggatgagcaggtgggtggacagcgtggacgagcgcttgaaggccttgccgcacatgcggcactcgaagctgcgctcctgccggaggaaatgaggccccggggggtcaggtgcaggctcaggactggacccggccgggatcccctgggagtggacgtgcgtgtgctgctccaggctcacagcgtggccgaaggttttgccgcagatgtcacaggcgaagggccgggtcccactatgggagcgtcgcacatgcacttcgagcccgtgaggggtggagaagaccttgttgcacttcacacagtggtacgcatccatgcctggggagtagcggaggctgaagtccaaggcgggctcagtgctgggcacaagaggactgccgtacaggctgacggagtgctccaggaaggctgactgcatggtggagggggcctgccggtagctgtggccataggttgtggccaaggtgtcccaggagaagctaggcttgtagaatgggggtgagtcggacagtggagagtccccatcctggggtcgggacagcacaatggggccctctggtgccggggccatcctggccaagttctggtcctgctccagctccggctctcgtttgaggttggtccagtccaggcactggtttgggaatagagtgctaaggacagggctgttgcttggagcctggtctctgggcaccggggtaagggcaggaggccagagcggttcatcttcctgcacacggggctggtggtaggtgtgagccttcttgctcttcaccaggaaggagcgtggcattttcagtgtgcaccccacacctgtccggagctgtccctcgcctgggttctgccggagcttcccgaggtgggaactgcaaagcctctctcgggactggcctccactctgtcaactgtgtgactctttgcacaaatagatacttctcctttttgctctgtctctctgtgtgtttttcctcttctgttcccctccctgattttcaatctgattatttgtgtcaaaatctggcggtgaacaagcagccaatgaagagagcgcgggagctcagccgtatttgcttatcaaaactttccaggacacaagacttcgaattctcatttctaaccctcgacacttggagcggcacgctttctctctgcagagaaattcagaatttcgctggaaattttgaataacatatttatagtggtactattcacaataggctggtcttgaactcctggcctcaagcgatcctcctgcctcagcctcccaaagtgctgggattacaggcacgagctgctgtgcccagccagggacacatcttgagtattctttaggacaaaaatctcagcttcagagatcaatactccgtgtttttcacaatgtcggcaccctttcaaataacagcacttttccagatgcgagttgcaggaagtttcaaaaagatggggtcttgctctgtagcccaggctggtcttgaactcctggtctcaagcaatcctcccaagctcctg

SEQ ID NO: 16670 - RNA, 1648 nt, Homo sapiens
  source 1..1648: mol_type = other RNA
gttttaccacctccaggagactggagatttgggcatgtgaggctggcctccaggtgacaggaccgcagggcaggctggccaggagctgggagccggcgcagcctcacttgagattgtgctggctctcgcggtgccgccgcaggtccaccttgcgctggaagcctttggtgcacagctcacagctgaagggcttgaagcctgtgtgcttgcggctgtgggtgatgaggttggagctctggctgaaggcctttccgcacacctggcacttgtgcggcttctcacctgtgtggatgtaggtgtgcttcttcatgtcggacttctggtggaaacgcttgccgcagaactggcaggggtagggccgcgtgtctgagtggatgagcaggtgggtggacagcgtggacgagcgcttgaaggccttgccgcacatgcggcactcgaagctgcgctcctgccggaggaaatgaggccccggggggtcaggtgcaggctcaggactggacccggccgggatcccctgggagtggacgtgcgtgtgctgctccaggctcacagcgtggccgaaggttttgccgcagatgtcacaggcgaagggccgggtcccactatgggagcgtcgcacatgcacttcgagcccgtgaggggtggagaagaccttgttgcacttcacacagtggtacgcatccatgcctggggagtagcggaggctgaagtccaaggcgggctcagtgctgggcacaagaggactgccgtacaggctgacggagtgctccaggaaggctgactgcatggtggagggggcctgccggtagctgtggccataggttgtggccaaggtgtcccaggagaagctaggcttgtagaatgggggtgagtcggacagtggagagtccccatcctggggtcgggacagcacaatggggccctctggtgccggggccatcctggccaagttctggtcctgctccagctccggctctcgtttgaggttggtccagtccaggcactggtttgggaatagagtgctaaggacagggctgttgcttggagcctggtctctgggcaccggggtaagggcaggaggccagagcggttcatcttcctgcacacggggctggtggtaggtgtgagccttcttgctcttcaccaggaaggagcgtggcattttcagtgtgcaccccacacctgtccggagctgtccctcgcctgggttctgccggagcttcccgaggtgggaactgcaaagcctctctcgggactggcctccactctgtcaactgtgtgactctttgcacaaatagatacttctcctttttgctctgtctctctgtgtgtttttcctcttctgttcccctccctgattttcaatctgattatttgtgtcaaaatctggcggtgaacaagcagccaatgaagagagcgcgggagctcagccgtatttgcttatcaaaactttccaggacacaagacttcgaattctcatttctaaccctcgacacttggagcggcacgctttctctctgcagagaaattcagaatttcgctggaaattttgaataacatcctgaggcttgtgagagccaggctggtgcaatgcccctagtacccgagccggccacatgcatagaggcccctcttgtccttgcagagg

SEQ ID NO: 16671 - RNA, 1608 nt, Homo sapiens
  source 1..1608: mol_type = other RNA
gttttaccacctccaggagactggagatttgggcatgtgaggctggcctccaggtgacaggaccgcagggcaggctggccaggagctgggagccggcgcagcctcacttgagattgtgctggctctcgcggtgccgccgcaggtccaccttgcgctggaagcctttggtgcacagctcacagctgaagggcttgaagcctgtgtgcttgcggctgtgggtgatgaggttggagctctggctgaaggcctttccgcacacctggcacttgtgcggcttctcacctgtgtggatgtaggtgtgcttcttcatgtcggacttctggtggaaacgcttgccgcagaactggcaggggtagggccgcgtgtctgagtggatgagcaggtgggtggacagcgtggacgagcgcttgaaggccttgccgcacatgcggcactcgaagctgcgctcctgccggaggaaatgaggccccggggggtcaggtgcaggctcaggactggacccggccgggatcccctgggagtggacgtgcgtgtgctgctccaggctcacagcgtggccgaaggttttgccgcagatgtcacaggcgaagggccgggtcccactatgggagcgtcgcacatgcacttcgagcccgtgaggggtggagaagaccttgttgcacttcacacagtggtacgcatccatgcctggggagtagcggaggctgaagtccaaggcgggctcagtgctgggcacaagaggactgccgtacaggctgacggagtgctccaggaaggctgactgcatggtggagggggcctgccggtagctgtggccataggttgtggccaaggtgtcccaggagaagctaggcttgtagaatgggggtgagtcggacagtggagagtccccatcctggggtcgggacagcacaatggggccctctggtgccggggccatcctggccaagttctggtcctgctccagctccggctctcgtttgaggttggtccagtccaggcactggtttgggaatagagtgctaaggacagggctgttgcttggagcctggtctctgggcaccggggtaagggcaggaggccagagcggttcatcttcctgcacacggggctggtggtaggtgtgagccttcttgctcttcaccaggaaggagcgtggcattttcagtgtgcaccccacacctgtccggagctgtccctcgcctgggttctgccggagcttcccgaggtgggaactgcaaagcctctctcgggactggcctccactctgtcaactgtgtgactctttgcacaaatagatacttctcctttttgctctgtctctctgtgtgtttttcctcttctgttcccctccctgattttcaatctgattatttgtgtcaaaatctggcggtgaacaagcagccaatgaagagagcgcgggagctcagccgtatttgcttatcaaaactttccaggacacaagacttcgaattctcatttctaaccctcgacacttggagcggcacgctttctctctgcagagaaattcagaatttcgctggaaattttgaataacatctttgagcgggtagaggcaccctggaggtgtggcagtgagttcggagg

SEQ ID NO: 16672 - RNA, 1264 nt, Homo sapiens
  source 1..1264: mol_type = other RNA
gttttaccacctccaggagactggagatttgggcatgtgaggctggcctccaggtgacaggaccgcagggcaggctggccaggagctgggagccggcgcagcctcacttgagattgtgctggctctcgcggtgccgccgcaggtccaccttgcgctggaagcctttggtgcacagctcacagctgaagggcttgaagcctgtgtgcttgcggctgtgggtgatgaggttggagctctggctgaaggcctttccgcacacctggcacttgtgcggcttctcacctgtgtggatgtaggtgtgcttcttcatgtcggacttctggtggaaacgcttgccgcagaactggcaggggtagggccgcgtgtctgagtggatgagcaggtgggtggacagcgtggacgagcgcttgaaggccttgccgcacatgcggcactcgaagctgcgctcctgggagtggacgtgcgtgtgctgctccaggctcacagcgtggccgaaggttttgccgcagatgtcacaggcgaagggccgggtcccactatgggagcgtcgcacatgcacttcgagcccgtgaggggtggagaagaccttgttgcacttcacacagtggtacgcatccatgcctggggagtagcggaggctgaagtccaaggcgggctcagtgctgggcacaagaggactgccgtacaggctgacggagtgctccaggaaggctgactgcatggtggagggggcctgccggtagctgtggccataggttgtggccaaggtgtcccaggagaagctaggcttgtagaatgggggtgagtcggacagtggagagtccccatcctggggtcgggacagcacaatggggccctctggtgccggggccatcctggccaagttctggtcctgctccagctccggctctcgtttgaggttggtccagtccaggcactggtttgggaatagagtgctaaggacagggctgttgcttggagcctggtctctgggcaccggggtaagggcaggaggccagagcggttcatcttcctgcacacggggctggtggtaggtgtgagccttcttgctcttcaccaggaaggagcgtggcattttcagtgtgcaccccacacctgtccggagctgtccctcgcctgggttctgccggagcttcccgaggtgggaactgcaaagcctctctcgggactggcctccactctgtcaactgtgtgactctttgcacaaatagatacttctcctttttgctctgtctctctgtgt

SEQ ID NO: 16673 - RNA, 1935 nt, Homo sapiens
  source 1..1935: mol_type = other RNA
gttttaccacctccaggagactggagatttgggcatgtgaggctggcctccaggtgacaggaccgcagggcaggctggccaggagctgggagccggcgcagcctcacttgagattgtgctggctctcgcggtgccgccgcaggtccaccttgcgctggaagcctttggtgcacagctcacagctgaagggcttgaagcctgtgtgcttgcggctgtgggtgatgaggttggagctctggctgaaggcctttccgcacacctggcacttgtgcggcttctcacctgtgtggatgtaggtgtgcttcttcatgtcggacttctggtggaaacgcttgccgcagaactggcaggggtagggccgcgtgtctgagtggatgagcaggtgggtggacagcgtggacgagcgcttgaaggccttgccgcacatgcggcactcgaagctgcgctcctgggagtggacgtgcgtgtgctgctccaggctcacagcgtggccgaaggttttgccgcagatgtcacaggcgaagggccgggtcccactatgggagcgtcgcacatgcacttcgagcccgtgaggggtggagaagaccttgttgcacttcacacagtggtacgcatccatgcctggggagtagcggaggctgaagtccaaggcgggctcagtgctgggcacaagaggactgccgtacaggctgacggagtgctccaggaaggctgactgcatggtggagggggcctgccggtagctgtggccataggttgtggccaaggtgtcccaggagaagctaggcttgtagaatgggggtgagtcggacagtggagagtccccatcctggggtcgggacagcacaatggggccctctggtgccggggccatcctggccaagttctggtcctgctccagctccggctctcgtttgaggttggtccagtccaggcactggtttgggaatagagtgctaaggacagggctgttgcttggagcctggtctctgggcaccggggtaagggcaggaggccagagcggttcatcttcctgcacacggggctggtggtaggtgtgagccttcttgctcttcaccaggaaggagcgtggcattttcagtgtgcaccccacacctgtccggagctgtccctcgcctgggttctgccggagcttcccgaggtgggaactgcaaagcctctctcgggactggcctccactctgtcaactgtgtgactctttgcacaaatagatacttctcctttttgctctgtctctctgtgtgtttttcctcttctgttcccctccctgattttcaatctgattatttgtgtcaaaatctggcggtgaacaagcagccaatgaagagagcgcgggagctcagccgtatttgcttatcaaaactttccaggacacaagacttcgaattctcatttctaaccctcgacacttggagcggcacgctttctctatttatagtggtactattcacaataggctggtcttgaactcctggcctcaagcgatcctcctgcctcagcctcccaaagtgctgggattacaggcacgagctgctgtgcccagccagggacacatcttgagtattctttaggacaaaaatctcagcttcagagatcaatactccgtgtttttcacaatgtcggcaccctttcaaataacagcacttttccagatgcgagttgcaggaagtttcaaaaagatggggtcttgctctgtagcccaggctggtcttgaactcctggtctcaagcaatcctcccaagctcctgagtagctttcctcgaacaaaaaccagcctgatgcctactccttcaaaatgcctttcatatcccacagttcgacttcatctcactctgcctcctctcacagggctttgtgttcgtgctggatggagcccatcatactcagcctcgcaataaaggccacctatctagt

SEQ ID NO: 16674 - RNA, 1812 nt, Homo sapiens
  source 1..1812: mol_type = other RNA
gttttaccacctccaggagactggagatttgggcatgtgaggctggcctccaggtgacaggaccgcagggcaggctggccaggagctgggagccggcgcagcctcacttgagattgtgctggctctcgcggtgccgccgcaggtccaccttgcgctggaagcctttggtgcacagctcacagctgaagggcttgaagcctgtgtgcttgcggctgtgggtgatgaggttggagctctggctgaaggcctttccgcacacctggcacttgtgcggcttctcacctgtgtggatgtaggtgtgcttcttcatgtcggacttctggtggaaacgcttgccgcagaactggcaggggtagggccgcgtgtctgagtggatgagcaggtgggtggacagcgtggacgagcgcttgaaggccttgccgcacatgcggcactcgaagctgcgctcctgggagtggacgtgcgtgtgctgctccaggctcacagcgtggccgaaggttttgccgcagatgtcacaggcgaagggccgggtcccactatgggagcgtcgcacatgcacttcgagcccgtgaggggtggagaagaccttgttgcacttcacacagtggtacgcatccatgcctggggagtagcggaggctgaagtccaaggcgggctcagtgctgggcacaagaggactgccgtacaggctgacggagtgctccaggaaggctgactgcatggtggagggggcctgccggtagctgtggccataggttgtggccaaggtgtcccaggagaagctaggcttgtagaatgggggtgagtcggacagtggagagtccccatcctggggtcgggacagcacaatggggccctctggtgccggggccatcctggccaagttctggtcctgctccagctccggctctcgtttgaggttggtccagtccaggcactggtttgggaatagagtgctaaggacagggctgttgcttggagcctggtctctgggcaccggggtaagggcaggaggccagagcggttcatcttcctgcacacggggctggtggtaggtgtgagccttcttgctcttcaccaggaaggagcgtggcattttcagtgtgcaccccacacctgtccggagctgtccctcgcctgggttctgccggagcttcccgaggtgggaactgcaaagcctctctcgggactggcctccactctgtcaactgtgtgactctttgcacaaatagatacttctcctttttgctctgtctctctgtgtgtttttcctcttctgttcccctccctgattttcaatctgattatttgtgtcaaaatctggcggtgaacaagcagccaatgaagagagcgcgggagctcagccgtatttgcttatcaaaactttccaggacacaagacttcgaattctcatttctaaccctcgacacttggagcggcacgctttctctctgcagagaaattcagaatttcgctggaaattttgaataacatatttatagtggtactattcacaataggctggtcttgaactcctggcctcaagcgatcctcctgcctcagcctcccaaagtgctgggattacaggcacgagctgctgtgcccagccagggacacatcttgagtattctttaggacaaaaatctcagcttcagagatcaatactccgtgtttttcacaatgtcggcaccctttcaaataacagcacttttccagatgcgagttgcaggaagtttcaaaaagatggggtcttgctctgtagcccaggctggtcttgaactcctggtctcaagcaatcctcccaagctcctg

SEQ ID NO: 16675 - RNA, 1520 nt, Homo sapiens
  source 1..1520: mol_type = other RNA
gttttaccacctccaggagactggagatttgggcatgtgaggctggcctccaggtgacaggaccgcagggcaggctggccaggagctgggagccggcgcagcctcacttgagattgtgctggctctcgcggtgccgccgcaggtccaccttgcgctggaagcctttggtgcacagctcacagctgaagggcttgaagcctgtgtgcttgcggctgtgggtgatgaggttggagctctggctgaaggcctttccgcacacctggcacttgtgcggcttctcacctgtgtggatgtaggtgtgcttcttcatgtcggacttctggtggaaacgcttgccgcagaactggcaggggtagggccgcgtgtctgagtggatgagcaggtgggtggacagcgtggacgagcgcttgaaggccttgccgcacatgcggcactcgaagctgcgctccttgttgcacttcacacagtggtacgcatccatgcctggggagtagcggaggctgaagtccaaggcgggctcagtgctgggcacaagaggactgccgtacaggctgacggagtgctccaggaaggctgactgcatggtggagggggcctgccggtagctgtggccataggttgtggccaaggtgtcccaggagaagctaggcttgtagaatgggggtgagtcggacagtggagagtccccatcctggggtcgggacagcacaatggggccctctggtgccggggccatcctggccaagttctggtcctgctccagctccggctctcgtttgaggttggtccagtccaggcactggtttgggaatagagtgctaaggacagggctgttgcttggagcctggtctctgggcaccggggtaagggcaggaggccagagcggttcatcttcctgcacacggggctggtggtaggtgtgagccttcttgctcttcaccaggaaggagcgtggcattttcagtgtgcaccccacacccacggcgattctgcagacctcctcttcacaagtcctgttttagagtgagcatgtctcctcagatgcctcaacacttaaacttggttttttttctccaaaaataggtggaaagggctaacaacagccacagggaaaggcgagctgaaacagtacctctccatggtcggtcctattgttcctggagcctgggcagtgtgtgggagagggcagccctgtcatctccccttagtaggctctggaggggagagcgcctgactctcaaagtgtcctgggaatttggctgggcgcagtggctaatgcctgtaatcccaacactttgggaggctgaggcaggtggatcgtttgaggtcaagagttcgagaccagcctggccaacatggtgaaacccgtctctactaaaaatacaaaaattagccaggcgtggtaacacgcgcctgtaatcccagctacttgggaggctgaggcaggagaatcgcttgaattcgggaggcagaggtttcagtgcaatcgcaccactgcgctccagagtctcactctgtct

SEQ ID NO: 16676 - RNA, 1126 nt, Homo sapiens
  source 1..1126: mol_type = other RNA
gttttaccacctccaggagactggagatttgggcatgtgaggctggcctccaggtgacaggaccgcagggcaggctggccaggagctgggagccggcgcagcctcacttgagattgtgctggctctcgcggtgccgccgcaggtccaccttgcgctggaagcctttggtgcacagctcacagctgaagggcttgaagcctgtgtgcttgcggctgtgggtgatgaggttggagctctggctgaaggcctttccgcacacctggcacttgtgcggcttctcacctgtgtggatgtaggtgtgcttcttcatgtcggacttctggtggaaacgcttgccgcagaactggcaggggtagggccgcgtgtctgagtggatgagcaggtgggtggacagcgtggacgagcgcttgaaggccttgccgcacatgcggcactcgaagctgcgctccttgttgcacttcacacagtggtacgcatccatgcctggggagtagcggaggctgaagtccaaggcgggctcagtgctgggcacaagaggactgccgtacaggctgacggagtgctccaggaaggctgactgcatggtggagggggcctgccggtagctgtggccataggttgtggccaaggtgtcccaggagaagctaggcttgtagaatgggggtgagtcggacagtggagagtccccatcctggggtcgggacagcacaatggggccctctggtgccggggccatcctggccaagttctggtcctgctccagctccggctctcgtttgaggttggtccagtccaggcactggtttgggaatagagtgctaaggacagggctgttgcttggagcctggtctctgggcaccggggtaagggcaggaggccagagcggttcatcttcctgcacacggggctggtggtaggtgtgagccttcttgctcttcaccaggaaggagcgtggcattttcagtgtgcaccccacacctgtccggagctgtccctcgcctgggttctgccggagcttcccgaggtgggaactgcaaagcctctctcgggactggcctccactctgtcaactgtgtgactctttgcacaaatagatacttctcctttttgctctgtctctctgtgt

SEQ ID NO: 16677 - RNA, 1674 nt, Homo sapiens
  source 1..1674: mol_type = other RNA
gttttaccacctccaggagactggagatttgggcatgtgaggctggcctccaggtgacaggaccgcagggcaggctggccaggagctgggagccggcgcagcctcacttgagattgtgctggctctcgcggtgccgccgcaggtccaccttgcgctggaagcctttggtgcacagctcacagctgaagggcttgaagcctgtgtgcttgcggctgtgggtgatgaggttggagctctggctgaaggcctttccgcacacctggcacttgtgcggcttctcacctgtgtggatgtaggtgtgcttcttcatgtcggacttctggtggaaacgcttgccgcagaactggcaggggtagggccgcgtgtctgagtggatgagcaggtgggtggacagcgtggacgagcgcttgaaggccttgccgcacatgcggcactcgaagctgcgctccttgttgcacttcacacagtggtacgcatccatgcctggggagtagcggaggctgaagtccaaggcgggctcagtgctgggcacaagaggactgccgtacaggctgacggagtgctccaggaaggctgactgcatggtggagggggcctgccggtagctgtggccataggttgtggccaaggtgtcccaggagaagctaggcttgtagaatgggggtgagtcggacagtggagagtccccatcctggggtcgggacagcacaatggggccctctggtgccggggccatcctggccaagttctggtcctgctccagctccggctctcgtttgaggttggtccagtccaggcactggtttgggaatagagtgctaaggacagggctgttgcttggagcctggtctctgggcaccggggtaagggcaggaggccagagcggttcatcttcctgcacacggggctggtggtaggtgtgagccttcttgctcttcaccaggaaggagcgtggcattttcagtgtgcaccccacacctgtccggagctgtccctcgcctgggttctgccggagcttcccgaggtgggaactgcaaagcctctctcgggactggcctccactctgtcaactgtgtgactctttgcacaaatagatacttctcctttttgctctgtctctctgtgtgtttttcctcttctgttcccctccctgattttcaatctgattatttgtgtcaaaatctggcggtgaacaagcagccaatgaagagagcgcgggagctcagccgtatttgcttatcaaaactttccaggacacaagacttcgaattctcatttctaaccctcgacacttggagcggcacgctttctctctgcagagaaattcagaatttcgctggaaattttgaataacatatttatagtggtactattcacaataggctggtcttgaactcctggcctcaagcgatcctcctgcctcagcctcccaaagtgctgggattacaggcacgagctgctgtgcccagccagggacacatcttgagtattctttaggacaaaaatctcagcttcagagatcaatactccgtgtttttcacaatgtcggcaccctttcaaataacagcacttttccagatgcgagttgcaggaagtttcaaaaagatggggtcttgctctgtagcccaggctggtcttgaactcctggtctcaagcaatcctcccaagctcctg

SEQ ID NO: 16678 - RNA, 2343 nt, Homo sapiens
  source 1..2343: mol_type = other RNA
taaaaactgcaattactttctcctggtttacccagcacacagatactcgctctcggcatccaaagcgctggtggcttcatccaggatgaggactggggggttccgcaccagagcccgggccatggccacccgctgcttctggccacctgacagctgggcgcccttctcccctgtctctgtgctgtagccgtcctggagttccatgatgaagccgtgggcattggccttctgtgcggcctccaccaccatctcgaaaggcacagtgggcaggccgtaggagatgttatccgtgatggagcgggcgaacagcacgggctcctggctcaccagggagatcacacggtgcaagtacttgtggtcgtaggcgctgatgggcttgccgtccagcagcacccggcccccctccagggggtagaagttctccaggatgttgacacaggagctcttcccactgcccgagggccccaccagggccgtcaccttgccgggggacaggctgaaggagacattctgcaggacctgggtgtggggccgagtgcggtaggtgaaggtcacattctcaaagtccacccggccctccaggtggtcgggggccaagctgccatcgtgcaccatggtcggctgccggtcgatgaactcgaacaccttctcagcagcccccactccctgcatcaggccactgtagacggagcccacggactccatacaatctcccaggacaaactcgtagatgatgaaggcgatgaggttgccgctggtcatctggcctgagatgacaaggtggcccccgtagtagaggatgctgacctggaccaccagcagtgtgagcccgctgccccagacgtagtacatgtaggcagctgcctccttcctgttcagcttgtacacctgctgcagcttccgcaggtacacctctgcctcctcctcctcattggcgaagctccggacagtcttcatggcactgatggtctcctccgccgtgttgctcgctctggccagggcattctggacctctttggagagcctcttgtagtacttgccgtagatgttggacaccatcatgatgatggggaagcccatgaaggtgaccaaggagagctgccatgagaggctgaacatgaagaccaccacgcccgtgaccttgactgtgttccgcaggaagacattgatgttctgggagaccaggtcgctgaccatggtggtgtccgaggtcaggcgggagatgaggtcccctgtgcggttctcatcaaagaagcttgtctcctgggacaccagtgagcggaagagacagtttcgaaggcgaatgttcagtctggcaaatatgagggtaaaaatgccgccccgaatacctgcggcaaatgagctgccaatggccagcaggcacacgatgacgacagccgtgctgaactgatccatgcttttctggatgacgatgccatcaatggcgcggcccgtgtagtagggcaggaaggtctctcccagagctgccacgatgaggaagaaggaggcggccacgaggaaggccacgtcgggcttggtgtaggagagcagcttctgcagcgtggccccagacgcctgctcgggcggtggccggccgctcccagggaagccctcagcctcggtggccgcccctggctccagggcctgggtgcctggccgcacggtggacagcagccaccagagcaggaaggatgcgccgagtgaaatgtacgtccacacgaacagggcccaaaaccaggggtcccggatgggcctgcgcacctctgagaagagcagcagcttcaccatggcatagatgcccacgaagaggcacacgagggtgatgaccagccacgaggcccgcagccgccggggccccagcgcactgttcttggccacaccaatggtggctcccagcagcaggcagctgcggtacaggcaggctgcccagagatccagcaccgagtcaaagatgttgaagtggcggatgtcctccaggaggctgcggtccaggtggctgaagacatagatggccgtggtcacgcagatgtccacactcatgaaggccaaagtcaccaccaccgccttccacagccgcatcctgctggttggaggtgggcgggtgctgaaggccaggttgtagctcacgggggcaaggccatcatcatccacagggcgaggccaggcctgttacctggcaccaggtgagctctgggagggggcgcgcagcaggctcgggtctggggtgcagtttccgcgctgctcattgaagactgcgccggacgcggtcctcgctccgctcttcccgctgctcctccccgcctcccacccgcgctgcgccgctgcaaggtcggagctgagact

SEQ ID NO: 16679 - RNA, 28 nt, Homo sapiens
  source 1..28: mol_type = other RNA
taaaaactgcaattacttttacaccaat

SEQ ID NO: 16680 - RNA, 10926 nt, Homo sapiens
  source 1..10926: mol_type = other RNA
taaaacccacaattatgtttgtctagtagaaatatatctgctggaacactttggagaacagattggtaattttgccattacactagacattagccctttcaaagcagactaagagtacgtagttccttagtgaatacaaggcttcacaactgaagagcattgcagggagcttggctaaggtgaaaagggacttgctggagaggtacagcagaatgggatgggattagaaaacaacaatctattaggaaagatgaaaggaaggaattccccagtgttcacgctgagaagtcttcatattggaccagtgtgagggggtcttttatactgaggttttaaaaacctgacttcattttgtcctgaatgtagaagtgaagaaggacactagtttcaggcacctgggatggtggaaaagtttattcaactgaggctttccatgcattgggttgaatagctgagggaagctgaagactcttatctgaaaatatgatctgaaaatatttattgtataggaagacagaatgcctgatttctgaagttttcttgatggcccaactaaagaagaaaggcaccaaatcctcactttaacaggtaaatggagatcctgagggctggatacccaagagccaccattttacggattcctcagatttaaaaatgtctcagatagatatttccaaattctatttctattagcctctgtggataaagagttcctgaaactctggttttactttttttggaaaaaaaaaaaaaaaaaaaaaaaaaaaacaactcccaggaaaatgaacactatattgccaagctgcctccagggaaaggttgaagactagttaaaataattctaagcgtattgaaaaaagaaagtgtaaagatccagtattaaaatgaatgtttgagaatacagtggggacaactaggtaattcactgtcttacgcttttcagaagactggccctttgaaacgcagcctgttattgttggtcagatcatgtggcacttaagtagccccttggtcatatttttaaaagcaaatatagacagtgacagtcctacaggggaaaatcacagatacattcatatgcacctcttttgttcttcagatattgagtgggtcagctaaacaagatcactttgaatatgaacctctttgtattagtcacaccaacaaaaaagtttcaaaaaaagttttcactttcctacatttgctaagtctgagctttaaaaaattctaaaatcctctaaagacaatactgaagctgataatataaaaagcaaattagagcactaatgattattactagatgcaccagattaactgcagcaggttggtgatgggtgatataagcaaagacataatatttcaatcaactcatgatcataggcagattcaaaagttaaaatgaatataatgtaatatatatttcaatatagagttgttatatataatgtgtatgtcctaggtttcagaaatactgcaatgtagtgtattgtagttaagtaagcatacctaaatagtaactcatattctttcacaaagtcactagtactgttaattaaaggaaaaaataaaaccgaaacaactaattgtttttccagtaaaaagaaatacctatggttacagttacagacttcttttggatatagaaagacaatatacattttaaaaagtaataacgacaaaaaagttgcaactgtaagtagccttacttaacaggggaaggggaaaagtcaccagaatagaagaggaaagaaaatgtcctctgacttctgtaaaacagaaataatgtacaaatcataaaaaataacaaaccatctagtaaaagaagggcatgggagtgagaaaactgaatcctgaattccaggccaccaaaccctcagagtccattcattcagtatattatactagagtggcattctacttcaatgcttgagatgggcaagagcaatcaattcctacagattaccaaaaaacattccccccaacagtctattggtttgctagacatggtaaacaacccactcctggaaagactttggcaaaggccacattggtttcaggagacacagtttgtgaattacgatgatatcttgtgagtacaggcagaattaggaagctttagtttgagaataaaatttatgtgtgtgtgtgtgtgtgtgtgtgtgtgtgtgcacactgcattgcatagaggaaaggaatgaagacctttgagctatgggatggctcaggccaaagtttgtgtgggctttgcctgcctggcattggtccccacccctgccacctccaggagacctggggagacgccctggactgctgctccctcttgtctgctcaccagttgaagacttctgttataccttattatggaggaaaacagcctgtccctgtgggtttgctgtggattcaacaagctgcatttgtttctcccaattctgaaacattacaaaaagcaacagagtgggcaggtgactgcttcctgggaagggagccacaagtcttaaacacaatggtgggaagaggcaactgtatctatgcacgaggacctctgcctgtgtgtgcttcctttggggggcacacacacttccagatgacaataagtatatacacaaacacacacatgtgcacacatgtcaataaatccaatagaactgtagagtttgttaaatgcactctactccacataagcatattcaagtttctcatgaaacggatacatagaaattactgatggttgggctccttcagaatgccctaaagtctcatcacagatactgatgcacccaactaaggcaacaaagcataagcagatacgtgagatatgtcagaccttcgacttctaaccagaagttcaaaaatgtatcttgttgtcactgggcaatatgaatgtgaaacagttttgtgctgagggaagctcacactgtgtgtgcacatgtataaataatgtatactcatttatagacattttggacagcagcggtgacatactggatgggttaagactctttcattattagaatctacatataaattgcaatgagtttgctgggtaaaaacaactgttgcaacactagtagaaacagatgcccccaaggtttttttttttttttttttttttttctctcttggatgtatcaaaatctcattgaggcattctaaaccaaagaaacctctgaatttgaaacagggttagtagggacttttatacccagctgggcatcccagaagcctggactctcaggactgtggctagattttgcccatgatctgtagattatgctcttgcaccggagacttgaaagttatgagtttgcattcaaacaaagaaccaccagataaaacagatgttctctaaaactgaggaaaaaaagtttagagatatacactgtatagagaaagaaagctttttgctggattgttctccttgttaaggaaatgtttaaaactagtactcccgggcacctgtgattgcattttataggattctatttagtaatatgatgtctattttacattcagccccaacctacgtcactgaaatagaataggaaatagcagccactatctgagagtacccagttctaggaaagtttggtgcctcctcaagaagtcactatttccatagtcctcaatcatgaatagggcttgtttttgtgataatgtaactattaaacagcaagaaatgcctataacttcagagccttctcatttctatatcttttatcctcttcccagggctttctgatttaaggcaataatgctacactataagtagccttttgtgaaaataccttaattgaggtcacttaagattagatttcagtctgaaagtctacagtttacggagcaaaaggtggagcctaaagaaaccactggcaggtgttttagtcagtggtgtggaaagataatgtttcttgtttcaacccagggcatttttacccatcatgcagtgaggagaaaatacatagttctgaaaaagaacccacactaggtagccctaattttctatctcttcactctaaaaaggatggaaacaagccctactgttccataaccattcccagggatcggctaaggtacattgctgactgctatagactcagtgttcaaggagaaaaaaatcttcagagacttagaaaactctttgcaatattttggtcaggctgatcgtcttgatactcagtgctagaaatgatgctttggattagtagtttccacattctgaatttataggaacactgagtcaccacagccttttttcttgtaaaggtttaagtgatatcagaaatagcaactctacacggaaagcccttgggaatatgaaaatactctctctcaagagcaagggctcttccgtgccccttttctgcctctgtatgtagcctgagcaccagggtagagattgcttttgaaagtttgccccatgtaatctatttcctggctacctaagagaacagccgttttcttcatgaaaacacaaagaggggaaagaggctgctgctgttccagtgggaagttatgtctagccccagaaggcctggtggctgggtcagctcaagcactctcttcatgcactgcaggctcaggaggcattgggttgctttgctttttctatggaattagggagcctattgaaattctagtgcacccctccttttgtttgtcaccaagtcacatggttctgtcttcagtatcctatttttctttttttttaatttctttttctgaggaacaaaattggccatttaaataaagttcttttctagtgagtaaagaggtttctcagagccagaaatcactgaaaagagagtctgtcgaccctgcccatggaaaagcccagagatttctctaaccacttcttgccaaacttcctagttttgtgattggatgtttcttggtttagcattgtttggtgctgaatacattttgcaattcttttgttctctgccctagagcttccattaccctggacttcaactcattaccaaattaaagaattcttttagaagatttcttttaagagtcaggtcacaacagaaagggcgccctcctgttctcctaaatctcaagggcatctcaggttgtgtctgctcttacgttgcaccttccttttgttcccttttaatgcagcagcacactggctatagcagaggcagacctgatttgattatctgataccttttccacaaaatcatatatcccctgctcccagccccaactaatcaaataacatcttctagaacaacagaggaaagctccagaatgggtgtatatcctgtgactcctggccagatccaccttgctccctgtcttcctaggggtcacaggtgttgggagcattgtggaggagccccaacaaggaagcaacatatggctttattatgttttctcaggaatcgaaggggttttataaggggcatatctcatttttgacttctgtgctgagagaaaatattgagttttgggcgcaggcagagcacagacaggacagctggtgttcctgtgtgagggaagtacacatagctcaaggctttaggactgaatgtgaaacaaacatacctggaggaaaacttttttcattatcagaattcacaaattcttactgttcatgggttgaaaaagagtatttgggaccttatagaatattttgatgatacaaaataaaacccttatgacttttaaacacagcaaacccaagtctttctaaggccaagagctactatgatctctaagatgactaggaatgaactgaggctagaatatgagcaggaaattatccagcacacttaatcatggcacaaatagattcaaagcattaggaatttgggaagagaacggtctataaaactgttattaggagctaaagtttacctctcaattaaaagatacaggaaaccattttgatacagagattttcatttcagattttttttctttgcttagcttgtttccccctgtgtagaattgtaacagatccatgtgttccaattattttcttttttaggattatatttcacacatttgggggccttttttgtacaaatattggcatgtaataaggaaaaattgcccatgatgctgagataataccagtgtttttagtggtagaaaatattatttttttataaaccatatctaaatatcttgagataaaaattcccctttgactttttttcctctcccttgtttggcaaattccattttaaaattataaattgctaaaaaatgtcctttccatactatttctctcttccttgtactcatcctaagaagtcttaaatctggaacatttgcttttatcttatctatctgtttcctggctactagaaagaaatttttttagcactcatatcaccctaccatgaaggtctaaatgtaagatgactgtaggacttgaaacaaaaaaaaattaaaaagatccacactcattctttgattttgaagcaaatgtctttccctatttctaaagatatttgtgattgtttaacttaaaagtgagaattgacaatctaaaagcatctctatccttttgaaacaggtccagattggtttatttcctaaaatgtgggtcagtttggaaagtggccatttgatgggccaggaacatagcaataaacaactacctctttgctcctccagattagatctcccactccaatccagcttcttcctctttccacaaaataatttgtcaactattttagaatgtgacatatttgggaaggataaatgtacagtaggaatatgtctactgctatgcaaacctggctggtccattttgtcatggactacaatgattatatcacctcattaagaattctttagggatcctccacctcctcccccactcccttttttttaagagacacttcctttacagggaaaggatgatagactcctcagggtttcaagtcacctgcagctttttctctacatgttctaccaaaagaaaaggtggattctaacccaattgcttagcattttacatggcaaatcagcattaaggcaaatgggtctctctcagatttgagaaacagaaagctacacgtggcccataatggcacctaagatcaacttttcaggcggtattagtgaaaattcttcctactttgctaaatttgaacaaagacactttcaaatctactgtgaaacagtttaaaatattttaaagtggcttttggccttctttcatttgtaacatgtattgagtgatttcatgtcattgtctcctagctttaagagtttttttcttaaggtcaatcttctcttttcattttatgggtggaatcacttgttttccaaaatatcaaaacaattccatgacatagttaattaatgctccctctattggtggtaagtggaaatattagtcttacaacactgctattttaaaaagcaaaattagcaatagaaaaatgaacttactttatctcggaagctgttcctcactaactgttaaaacagatcagttttggacatacagttcttggcaggactcctcttagaaatcacaataggttacacttaatagtcagttaaccacccaagtttacattaaaacttctagcaaaatatccactgaattaagcactgtgggaccaaatcaaactcacaaacacttcagttacactaaccttacaaagcatcacaaagaacttatgaaaaagatccaagttaaccaaatgtctaaaatatatgaataaaaccaatttagtcattacagagttgtttgtgttggaagattttccctcgtttgctgcacagtttttgtaaataaaatgctgacaggaaaattagaaggaaaattaaattaaaatgtaatgtaattttgaaactaaaatacgctctcctttcttctttttaaaactgtagtttggtgttttgctttgtttaaagatttgctttcccctaagtatgttaaaatatgcccagcaatgaaatcactttgggagtttcagctaggtttaagaattcctatatttgagctggaatcccttcaggacactgtctataatgaaaatgtctctattataacaccttgatcaggaccgaggagagaaatccctactaggaagagagagtggcatctggtatgatgcaatagattggtggtcttttgaatggtggctgttggcatctgggaatttttttgttaatttccctaaaacctttcgaagaagcaagggttaattcgtcatctaaagaatgatcatcttattcagccctcttaaccatggtggaaacagtcagaaggtgatatttggaaggaaaaaagtaattttggcatcaatgcatcttgatctataacaggcttctcataatgatgctctttgtagttgggaagggtgaggagctatggcagagttttgtgaactcctcttcctggctgatcacaaaagaaaagaccccatttatcaagacttctagactattagtgtttcactaagaaaaaaagtaaagtcaatagaaattctagaattgtaagatctcaatgaaattttggagaagcaagcaatctctttctgaaagataaagtctcttccatgaaaaagaacagaattctagatgaatcagttgaaaaaattattcagtggggcaacttaagcttgctaaagtcaaagaactacatatcaaaatacaaagcagcaattcaaattacagcagggatgggctggccacagaggccctcatcaacccaggcaatacttaaaataataaaaattaagaaaaattaaaaaaaatatgaagaaaatatccttcctctctttcaaatataactttagttgccttttattctttctatctggaagcagtatcgctaaccttaacagtcttgacttaccaaaaaatatatatatgtgtgtgaaataaaataaaagagaaggaattggtggcagtgtatgcaaaaccaaaatgaaaaaaattacttttaacaatttcactttttttgtttttttttttacacaaatactgttgtaaatatattaaaaaaatcagcattctatctggtaaacgtcacttttgcccctctataaaattttgaattaaaaaagcctcaagaactttttattgttccccccaccctccatttctttttctttttctcttccacaagaatatatcctgacactttttttttttttgcaaagattgttggaaataatccttctcttgtacctagaaacataggtgcaaatttctgatatctttgttttatctgcattcctgcctttcatgaaagtccctcttgattgtgctgaggctgtggctcagcgaagacactgaataaatacgatagccactgttgcttgttgcttgtccaagtcttcctggcttctgctgcaagagggggatatggagaaggtgggccagggtgtgtggacccgggcagaatctggggaagaagcctgccattcgtctttctttcccacaccaccgaacccactgcccttcccacccccacagcccttttatgaaatcagacaacgtggtaggtggaaaacagcagggcctttcctctgggttttcaaccagaagtgatattccacagttttaactggttactgtgaagtccaagcggccagaattgtgaaaatgtccactgaaacactgcaagcggtgtacttaaagacagtaggccttttagattttgttatatattttttgtagtgctcttcacaagtggaaattttttttttttttttacttttttttaaaagatttttttgtaaagaagggttgtatttagaggccagtagctagagatccaaccagtggacctcttgaagcactaccaggccttaaggccaccatccgagggagactgggaaaactattattcacccaagcctccggaaatgtaatgtaccagcaggcaaaaaacagttcttcatgtagtacaaaatgaaacgaaacaaaaacaaaaacagaaagtaaaaatgaaaccaaaacatttcttaaattctagtgccatagcttttttgtttgtttgttttttgttgttgttttgttttgttcataagaaagagagaaagatactacttatccgtcagacacatgcatcctcatgtggtcgttgaactgctcgatttggtcaaactttgctgggcagacggagcagacgtaagtggtcccctccgtgcaggccaccacgcctggggggccagcgcgggcacctgggggtgtgcctgcagggggggtcccattgctggcactgtgcagggccacgtgtcgctccaggagggtcttgtgagagaacttctttttgcagatgtagcactcgtaggacttctctccccggtggaggcgcatgtgcacgttgagggagctcttctgggtgaagcgcttgttgcagatactacactggtatgccctcactcctgtgtgtgtcaccatgtgcttgataaggtaatcctttaaggagaaggagcgccaacagatgctgcattggtggggcttctcacaatcagatgacccggtgtgagcgtgagagtttgtcagtgaatgtgttgagtggatgagggctgggtctggagacaaaacagcttcaaagttcaggcagggaaggcccggcttggcgctggatccacccggctgagtaatctcattctcctcagatgccttctggttttcagctgtcttgggtttcttcagtagtttcaaaatcaatggtgtcactcttcaggtaaattactccaaggcttgggcctagtgcagatgttcattggggcagggagcagagagcggctgcatgtaaagagaaggggcaggtcacagactgatggtcaaagataggaatacagtgcagctcaatcttttgtttttaaggtgcagtgatttcagtctctaaatgtaacttcaggcagtctgtgcagctatggggcacaaacttgcaattcatcaattcatggcctctgaaactcaaatgctttc

SEQ ID NO: 16681 - RNA, 12933 nt, Homo sapiens
  source 1..12933: mol_type = other RNA
taaaacccacaattatgtttgtctagtagaaatatatctgctggaacactttggagaacagattggtaattttgccattacactagacattagccctttcaaagcagactaagagtacgtagttccttagtgaatacaaggcttcacaactgaagagcattgcagggagcttggctaaggtgaaaagggacttgctggagaggtacagcagaatgggatgggattagaaaacaacaatctattaggaaagatgaaaggaaggaattccccagtgttcacgctgagaagtcttcatattggaccagtgtgagggggtcttttatactgaggttttaaaaacctgacttcattttgtcctgaatgtagaagtgaagaaggacactagtttcaggcacctgggatggtggaaaagtttattcaactgaggctttccatgcattgggttgaatagctgagggaagctgaagactcttatctgaaaatatgatctgaaaatatttattgtataggaagacagaatgcctgatttctgaagttttcttgatggcccaactaaagaagaaaggcaccaaatcctcactttaacaggtaaatggagatcctgagggctggatacccaagagccaccattttacggattcctcagatttaaaaatgtctcagatagatatttccaaattctatttctattagcctctgtggataaagagttcctgaaactctggttttactttttttggaaaaaaaaaaaaaaaaaaaaaaaaaaaacaactcccaggaaaatgaacactatattgccaagctgcctccagggaaaggttgaagactagttaaaataattctaagcgtattgaaaaaagaaagtgtaaagatccagtattaaaatgaatgtttgagaatacagtggggacaactaggtaattcactgtcttacgcttttcagaagactggccctttgaaacgcagcctgttattgttggtcagatcatgtggcacttaagtagccccttggtcatatttttaaaagcaaatatagacagtgacagtcctacaggggaaaatcacagatacattcatatgcacctcttttgttcttcagatattgagtgggtcagctaaacaagatcactttgaatatgaacctctttgtattagtcacaccaacaaaaaagtttcaaaaaaagttttcactttcctacatttgctaagtctgagctttaaaaaattctaaaatcctctaaagacaatactgaagctgataatataaaaagcaaattagagcactaatgattattactagatgcaccagattaactgcagcaggttggtgatgggtgatataagcaaagacataatatttcaatcaactcatgatcataggcagattcaaaagttaaaatgaatataatgtaatatatatttcaatatagagttgttatatataatgtgtatgtcctaggtttcagaaatactgcaatgtagtgtattgtagttaagtaagcatacctaaatagtaactcatattctttcacaaagtcactagtactgttaattaaaggaaaaaataaaaccgaaacaactaattgtttttccagtaaaaagaaatacctatggttacagttacagacttcttttggatatagaaagacaatatacattttaaaaagtaataacgacaaaaaagttgcaactgtaagtagccttacttaacaggggaaggggaaaagtcaccagaatagaagaggaaagaaaatgtcctctgacttctgtaaaacagaaataatgtacaaatcataaaaaataacaaaccatctagtaaaagaagggcatgggagtgagaaaactgaatcctgaattccaggccaccaaaccctcagagtccattcattcagtatattatactagagtggcattctacttcaatgcttgagatgggcaagagcaatcaattcctacagattaccaaaaaacattccccccaacagtctattggtttgctagacatggtaaacaacccactcctggaaagactttggcaaaggccacattggtttcaggagacacagtttgtgaattacgatgatatcttgtgagtacaggcagaattaggaagctttagtttgagaataaaatttatgtgtgtgtgtgtgtgtgtgtgtgtgtgtgtgcacactgcattgcatagaggaaaggaatgaagacctttgagctatgggatggctcaggccaaagtttgtgtgggctttgcctgcctggcattggtccccacccctgccacctccaggagacctggggagacgccctggactgctgctccctcttgtctgctcaccagttgaagacttctgttataccttattatggaggaaaacagcctgtccctgtgggtttgctgtggattcaacaagctgcatttgtttctcccaattctgaaacattacaaaaagcaacagagtgggcaggtgactgcttcctgggaagggagccacaagtcttaaacacaatggtgggaagaggcaactgtatctatgcacgaggacctctgcctgtgtgtgcttcctttggggggcacacacacttccagatgacaataagtatatacacaaacacacacatgtgcacacatgtcaataaatccaatagaactgtagagtttgttaaatgcactctactccacataagcatattcaagtttctcatgaaacggatacatagaaattactgatggttgggctccttcagaatgccctaaagtctcatcacagatactgatgcacccaactaaggcaacaaagcataagcagatacgtgagatatgtcagaccttcgacttctaaccagaagttcaaaaatgtatcttgttgtcactgggcaatatgaatgtgaaacagttttgtgctgagggaagctcacactgtgtgtgcacatgtataaataatgtatactcatttatagacattttggacagcagcggtgacatactggatgggttaagactctttcattattagaatctacatataaattgcaatgagtttgctgggtaaaaacaactgttgcaacactagtagaaacagatgcccccaaggtttttttttttttttttttttttttctctcttggatgtatcaaaatctcattgaggcattctaaaccaaagaaacctctgaatttgaaacagggttagtagggacttttatacccagctgggcatcccagaagcctggactctcaggactgtggctagattttgcccatgatctgtagattatgctcttgcaccggagacttgaaagttatgagtttgcattcaaacaaagaaccaccagataaaacagatgttctctaaaactgaggaaaaaaagtttagagatatacactgtatagagaaagaaagctttttgctggattgttctccttgttaaggaaatgtttaaaactagtactcccgggcacctgtgattgcattttataggattctatttagtaatatgatgtctattttacattcagccccaacctacgtcactgaaatagaataggaaatagcagccactatctgagagtacccagttctaggaaagtttggtgcctcctcaagaagtcactatttccatagtcctcaatcatgaatagggcttgtttttgtgataatgtaactattaaacagcaagaaatgcctataacttcagagccttctcatttctatatcttttatcctcttcccagggctttctgatttaaggcaataatgctacactataagtagccttttgtgaaaataccttaattgaggtcacttaagattagatttcagtctgaaagtctacagtttacggagcaaaaggtggagcctaaagaaaccactggcaggtgttttagtcagtggtgtggaaagataatgtttcttgtttcaacccagggcatttttacccatcatgcagtgaggagaaaatacatagttctgaaaaagaacccacactaggtagccctaattttctatctcttcactctaaaaaggatggaaacaagccctactgttccataaccattcccagggatcggctaaggtacattgctgactgctatagactcagtgttcaaggagaaaaaaatcttcagagacttagaaaactctttgcaatattttggtcaggctgatcgtcttgatactcagtgctagaaatgatgctttggattagtagtttccacattctgaatttataggaacactgagtcaccacagccttttttcttgtaaaggtttaagtgatatcagaaatagcaactctacacggaaagcccttgggaatatgaaaatactctctctcaagagcaagggctcttccgtgccccttttctgcctctgtatgtagcctgagcaccagggtagagattgcttttgaaagtttgccccatgtaatctatttcctggctacctaagagaacagccgttttcttcatgaaaacacaaagaggggaaagaggctgctgctgttccagtgggaagttatgtctagccccagaaggcctggtggctgggtcagctcaagcactctcttcatgcactgcaggctcaggaggcattgggttgctttgctttttctatggaattagggagcctattgaaattctagtgcacccctccttttgtttgtcaccaagtcacatggttctgtcttcagtatcctatttttctttttttttaatttctttttctgaggaacaaaattggccatttaaataaagttcttttctagtgagtaaagaggtttctcagagccagaaatcactgaaaagagagtctgtcgaccctgcccatggaaaagcccagagatttctctaaccacttcttgccaaacttcctagttttgtgattggatgtttcttggtttagcattgtttggtgctgaatacattttgcaattcttttgttctctgccctagagcttccattaccctggacttcaactcattaccaaattaaagaattcttttagaagatttcttttaagagtcaggtcacaacagaaagggcgccctcctgttctcctaaatctcaagggcatctcaggttgtgtctgctcttacgttgcaccttccttttgttcccttttaatgcagcagcacactggctatagcagaggcagacctgatttgattatctgataccttttccacaaaatcatatatcccctgctcccagccccaactaatcaaataacatcttctagaacaacagaggaaagctccagaatgggtgtatatcctgtgactcctggccagatccaccttgctccctgtcttcctaggggtcacaggtgttgggagcattgtggaggagccccaacaaggaagcaacatatggctttattatgttttctcaggaatcgaaggggttttataaggggcatatctcatttttgacttctgtgctgagagaaaatattgagttttgggcgcaggcagagcacagacaggacagctggtgttcctgtgtgagggaagtacacatagctcaaggctttaggactgaatgtgaaacaaacatacctggaggaaaacttttttcattatcagaattcacaaattcttactgttcatgggttgaaaaagagtatttgggaccttatagaatattttgatgatacaaaataaaacccttatgacttttaaacacagcaaacccaagtctttctaaggccaagagctactatgatctctaagatgactaggaatgaactgaggctagaatatgagcaggaaattatccagcacacttaatcatggcacaaatagattcaaagcattaggaatttgggaagagaacggtctataaaactgttattaggagctaaagtttacctctcaattaaaagatacaggaaaccattttgatacagagattttcatttcagattttttttctttgcttagcttgtttccccctgtgtagaattgtaacagatccatgtgttccaattattttcttttttaggattatatttcacacatttgggggccttttttgtacaaatattggcatgtaataaggaaaaattgcccatgatgctgagataataccagtgtttttagtggtagaaaatattatttttttataaaccatatctaaatatcttgagataaaaattcccctttgactttttttcctctcccttgtttggcaaattccattttaaaattataaattgctaaaaaatgtcctttccatactatttctctcttccttgtactcatcctaagaagtcttaaatctggaacatttgcttttatcttatctatctgtttcctggctactagaaagaaatttttttagcactcatatcaccctaccatgaaggtctaaatgtaagatgactgtaggacttgaaacaaaaaaaaattaaaaagatccacactcattctttgattttgaagcaaatgtctttccctatttctaaagatatttgtgattgtttaacttaaaagtgagaattgacaatctaaaagcatctctatccttttgaaacaggtccagattggtttatttcctaaaatgtgggtcagtttggaaagtggccatttgatgggccaggaacatagcaataaacaactacctctttgctcctccagattagatctcccactccaatccagcttcttcctctttccacaaaataatttgtcaactattttagaatgtgacatatttgggaaggataaatgtacagtaggaatatgtctactgctatgcaaacctggctggtccattttgtcatggactacaatgattatatcacctcattaagaattctttagggatcctccacctcctcccccactcccttttttttaagagacacttcctttacagggaaaggatgatagactcctcagggtttcaagtcacctgcagctttttctctacatgttctaccaaaagaaaaggtggattctaacccaattgcttagcattttacatggcaaatcagcattaaggcaaatgggtctctctcagatttgagaaacagaaagctacacgtggcccataatggcacctaagatcaacttttcaggcggtattagtgaaaattcttcctactttgctaaatttgaacaaagacactttcaaatctactgtgaaacagtttaaaatattttaaagtggcttttggccttctttcatttgtaacatgtattgagtgatttcatgtcattgtctcctagctttaagagtttttttcttaaggtcaatcttctcttttcattttatgggtggaatcacttgttttccaaaatatcaaaacaattccatgacatagttaattaatgctccctctattggtggtaagtggaaatattagtcttacaacactgctattttaaaaagcaaaattagcaatagaaaaatgaacttactttatctcggaagctgttcctcactaactgttaaaacagatcagttttggacatacagttcttggcaggactcctcttagaaatcacaataggttacacttaatagtcagttaaccacccaagtttacattaaaacttctagcaaaatatccactgaattaagcactgtgggaccaaatcaaactcacaaacacttcagttacactaaccttacaaagcatcacaaagaacttatgaaaaagatccaagttaaccaaatgtctaaaatatatgaataaaaccaatttagtcattacagagttgtttgtgttggaagattttccctcgtttgctgcacagtttttgtaaataaaatgctgacaggaaaattagaaggaaaattaaattaaaatgtaatgtaattttgaaactaaaatacgctctcctttcttctttttaaaactgtagtttggtgttttgctttgtttaaagatttgctttcccctaagtatgttaaaatatgcccagcaatgaaatcactttgggagtttcagctaggtttaagaattcctatatttgagctggaatcccttcaggacactgtctataatgaaaatgtctctattataacaccttgatcaggaccgaggagagaaatccctactaggaagagagagtggcatctggtatgatgcaatagattggtggtcttttgaatggtggctgttggcatctgggaatttttttgttaatttccctaaaacctttcgaagaagcaagggttaattcgtcatctaaagaatgatcatcttattcagccctcttaaccatggtggaaacagtcagaaggtgatatttggaaggaaaaaagtaattttggcatcaatgcatcttgatctataacaggcttctcataatgatgctctttgtagttgggaagggtgaggagctatggcagagttttgtgaactcctcttcctggctgatcacaaaagaaaagaccccatttatcaagacttctagactattagtgtttcactaagaaaaaaagtaaagtcaatagaaattctagaattgtaagatctcaatgaaattttggagaagcaagcaatctctttctgaaagataaagtctcttccatgaaaaagaacagaattctagatgaatcagttgaaaaaattattcagtggggcaacttaagcttgctaaagtcaaagaactacatatcaaaatacaaagcagcaattcaaattacagcagggatgggctggccacagaggccctcatcaacccaggcaatacttaaaataataaaaattaagaaaaattaaaaaaaatatgaagaaaatatccttcctctctttcaaatataactttagttgccttttattctttctatctggaagcagtatcgctaaccttaacagtcttgacttaccaaaaaatatatatatgtgtgtgaaataaaataaaagagaaggaattggtggcagtgtatgcaaaaccaaaatgaaaaaaattacttttaacaatttcactttttttgtttttttttttacacaaatactgttgtaaatatattaaaaaaatcagcattctatctggtaaacgtcacttttgcccctctataaaattttgaattaaaaaagcctcaagaactttttattgttccccccaccctccatttctttttctttttctcttccacaagaatatatcctgacactttttttttttttgcaaagattgttggaaataatccttctcttgtacctagaaacataggtgcaaatttctgatatctttgttttatctgcattcctgcctttcatgaaagtccctcttgattgtgctgaggctgtggctcagcgaagacactgaataaatacgatagccactgttgcttgttgcttgtccaagtcttcctggcttctgctgcaagagggggatatggagaaggtgggccagggtgtgtggacccgggcagaatctggggaagaagcctgccattcgtctttctttcccacaccaccgaacccactgcccttcccacccccacagcccttttatgaaatcagacaacgtggtaggtggaaaacagcagggcctttcctctgggttttcaaccagaagtgatattccacagttttaactggttactgtgaagtccaagcggccagaattgtgaaaatgtccactgaaacactgcaagcggtgtacttaaagacagtaggccttttagattttgttatatattttttgtagtgctcttcacaagtggaaattttttttttttttttacttttttttaaaagatttttttgtaaagaagggttgtatttagaggccagtagctagagatccaaccagtggacctcttgaagcactaccaggccttaaggccaccatccgagggagactgggaaaactattattcacccaagcctccggaaatgtaatgtaccagcaggcaaaaaacagttcttcatgtagtacaaaatgaaacgaaacaaaaacaaaaacagaaagtaaaaatgaaaccaaaacatttcttaaattctagtgccatagcttttttgtttgtttgttttttgttgttgttttgttttgttcataagaaagagagaaagatactacttatccgtcagacacatgcatcctcatgtggtcgttgaactgctcgatttggtcaaactttgctgggcagacggagcagacgtaagtggtcccctccgtgcaggccaccacgcctggggggccagcgcgggcacctgggggtgtgcctgcagggggggtcccattgctggcactgtgcagggccacgtgtcgctccaggagggtcttgtgagagaacttctttttgcagatgtagcactcgtaggacttctctccccggtggaggcgcatgtgcacgttgagggagctcttctgggtgaagcgcttgttgcagatactacactggtatgccctcactcctgtgtgtgtcaccatgtgcttgataaggtaatcctttaaggagaaggagcgccaacagatgctgcattggtggggcttctcacctgtgtgtacgaacatgtgcttgacgtagttctgtttggcggtgaaagtcttgttgcagagagtgcactcataaggctttttttcgccttgcccactggctgtgctgtggcctgcggatgaggccaggggctgtggcgctggcagctgtgcagtaaaggtcgacagaccgggctgggacactgtcacaaactgggtctgctggcctgccaggggctgtggcaggctgaagaggaaaggcttggggccactgcccgcgggctgggtagtgaagagggctggcaggtaggtgttgccagctgtgccaatgacctgcgtgttgctggtcaaggtcagaggcatcctcaggttgctggtgagggtttctgtctggcgtaagtagagctgggtacttggcaatggctgcccgatggacgtgttgaccgaaggctgttgtaggacgctcttgtcggagctgttgctgacagtgataacagtgctgtccatctccacttcattgcttctctccggagaggaagcacctgtttctagctggtttgtctgcggaccaccctcagcgggggcttctgcagcctgctcgggttgggtgggttcagcctggctgtcccgcgccgccccaggcccaaactgctgctccaccgagtcaggctcggtgcctatggaggagctgacgcccgagtcgaagctttcacctttgggctcactctcggtgccctcggcctggtctgtgtcttccgtgcactcctcggattcgttgcgttccaggatctgcaccctttgctgcccgtagtagtcgtaatcgtcctccatctcctgcttgatgtggatgttgcccactagggtctggatgcgcacaggccggggctgcttgcggcagtgcgtggtctcgggggtggtggacaggtagcgctccatctgctgcgagcgctcatggatgcgtgtgatccagctggggtcttccatgtggtggtcgcggggcaggccgagcgcagtctcgtggtggctgaccactgcgccgctgtaaaaagagcgctcgccgctgccattctgcatggagcacgcgtagagtgccgagtagatcctgtccacgctgtgctgtgggtggctctgcaggtagcccgactccgtgtcgctgctctggcctgacgtgcctgactcgggagtgccccgcggcgtgtcctggcccgagtcctggatccccgggaacacatcgcccacgttctgtgacacgatgcgcgtgcactcgtcgatgactgttttgatctgcaggatgctggcggccgtgaggatctgcagagcttccgactgcgagacccgtagcacgccgctgtacatgaagtcaatgagcttttgcactgactgcactgacaccaccgacgggatctcgatgtcgctgtagccaagcagcagtttgtcctggaagaaggggctgccggctgccagcacgcagcggtgtgcgcgcagcatgctcccgtggatgcgcaccgttacgtcacagaagtggccacggttgcgctgctcgttgagggtctcgagcacggaattgctgaagttgtgaaggttgatgctgtgaatgcgctcggtcatccccttgcaactgatgtcacaatcagatgacccggtgtgagcgtgagagtttgtcagtgaatgtgttgagtggatgagggctgggtctggagacaaaacagcttcaaagttcaggcagggaaggcccggcttggcgctggatccacccggctgagtaatctcattctcctcagatgccttctggttttcagctgtcttgggtttcttcagtagtttcaaaatcaatggtgtcactcttcaggtaaattactccaaggcttgggcctagtgcagatgttcattggggcagggagcagagagcggctgcatgtaaagagaaggggcaggtcacagactgatggtcaaagatcagacagcaatgtcatgaggaatatcctgttagtaatgatgaaacattaggaatacagtgcagctcaatcttttgtttttaaggtgcagtgatttcagtctctaaatgtaacttcaggcagtctgtgcagctatggggcacaaacttgcaattcatcaattcttcagccttcagagtcccaaaggcaattcttaacacttctttttatttgtagtggcatggatgacggagcagaaatagagaattcttgattaaccaggagaagaatatcataggcatgggtgtgagatcaactggagattcaaggaagctaaagtgcccagaatgaactaatgttgtaatgtagactgtgagcagagataaaattccagaagccaaggagtgttgtacggtaagtcctggcagtgccttcttccccagcgctgagtttctcttcttataatcggtgtctccctggaagtacagtgtgagtggtaatgactgcctgcctccctaatgagtccattttcctgctcttgatgttgtgtatatacacacactgc

SEQ ID NO: 16682 - RNA, 12768 nt, Homo sapiens
  source 1..12768: mol_type = other RNA
taaaacccacaattatgtttgtctagtagaaatatatctgctggaacactttggagaacagattggtaattttgccattacactagacattagccctttcaaagcagactaagagtacgtagttccttagtgaatacaaggcttcacaactgaagagcattgcagggagcttggctaaggtgaaaagggacttgctggagaggtacagcagaatgggatgggattagaaaacaacaatctattaggaaagatgaaaggaaggaattccccagtgttcacgctgagaagtcttcatattggaccagtgtgagggggtcttttatactgaggttttaaaaacctgacttcattttgtcctgaatgtagaagtgaagaaggacactagtttcaggcacctgggatggtggaaaagtttattcaactgaggctttccatgcattgggttgaatagctgagggaagctgaagactcttatctgaaaatatgatctgaaaatatttattgtataggaagacagaatgcctgatttctgaagttttcttgatggcccaactaaagaagaaaggcaccaaatcctcactttaacaggtaaatggagatcctgagggctggatacccaagagccaccattttacggattcctcagatttaaaaatgtctcagatagatatttccaaattctatttctattagcctctgtggataaagagttcctgaaactctggttttactttttttggaaaaaaaaaaaaaaaaaaaaaaaaaaaacaactcccaggaaaatgaacactatattgccaagctgcctccagggaaaggttgaagactagttaaaataattctaagcgtattgaaaaaagaaagtgtaaagatccagtattaaaatgaatgtttgagaatacagtggggacaactaggtaattcactgtcttacgcttttcagaagactggccctttgaaacgcagcctgttattgttggtcagatcatgtggcacttaagtagccccttggtcatatttttaaaagcaaatatagacagtgacagtcctacaggggaaaatcacagatacattcatatgcacctcttttgttcttcagatattgagtgggtcagctaaacaagatcactttgaatatgaacctctttgtattagtcacaccaacaaaaaagtttcaaaaaaagttttcactttcctacatttgctaagtctgagctttaaaaaattctaaaatcctctaaagacaatactgaagctgataatataaaaagcaaattagagcactaatgattattactagatgcaccagattaactgcagcaggttggtgatgggtgatataagcaaagacataatatttcaatcaactcatgatcataggcagattcaaaagttaaaatgaatataatgtaatatatatttcaatatagagttgttatatataatgtgtatgtcctaggtttcagaaatactgcaatgtagtgtattgtagttaagtaagcatacctaaatagtaactcatattctttcacaaagtcactagtactgttaattaaaggaaaaaataaaaccgaaacaactaattgtttttccagtaaaaagaaatacctatggttacagttacagacttcttttggatatagaaagacaatatacattttaaaaagtaataacgacaaaaaagttgcaactgtaagtagccttacttaacaggggaaggggaaaagtcaccagaatagaagaggaaagaaaatgtcctctgacttctgtaaaacagaaataatgtacaaatcataaaaaataacaaaccatctagtaaaagaagggcatgggagtgagaaaactgaatcctgaattccaggccaccaaaccctcagagtccattcattcagtatattatactagagtggcattctacttcaatgcttgagatgggcaagagcaatcaattcctacagattaccaaaaaacattccccccaacagtctattggtttgctagacatggtaaacaacccactcctggaaagactttggcaaaggccacattggtttcaggagacacagtttgtgaattacgatgatatcttgtgagtacaggcagaattaggaagctttagtttgagaataaaatttatgtgtgtgtgtgtgtgtgtgtgtgtgtgtgtgcacactgcattgcatagaggaaaggaatgaagacctttgagctatgggatggctcaggccaaagtttgtgtgggctttgcctgcctggcattggtccccacccctgccacctccaggagacctggggagacgccctggactgctgctccctcttgtctgctcaccagttgaagacttctgttataccttattatggaggaaaacagcctgtccctgtgggtttgctgtggattcaacaagctgcatttgtttctcccaattctgaaacattacaaaaagcaacagagtgggcaggtgactgcttcctgggaagggagccacaagtcttaaacacaatggtgggaagaggcaactgtatctatgcacgaggacctctgcctgtgtgtgcttcctttggggggcacacacacttccagatgacaataagtatatacacaaacacacacatgtgcacacatgtcaataaatccaatagaactgtagagtttgttaaatgcactctactccacataagcatattcaagtttctcatgaaacggatacatagaaattactgatggttgggctccttcagaatgccctaaagtctcatcacagatactgatgcacccaactaaggcaacaaagcataagcagatacgtgagatatgtcagaccttcgacttctaaccagaagttcaaaaatgtatcttgttgtcactgggcaatatgaatgtgaaacagttttgtgctgagggaagctcacactgtgtgtgcacatgtataaataatgtatactcatttatagacattttggacagcagcggtgacatactggatgggttaagactctttcattattagaatctacatataaattgcaatgagtttgctgggtaaaaacaactgttgcaacactagtagaaacagatgcccccaaggtttttttttttttttttttttttttctctcttggatgtatcaaaatctcattgaggcattctaaaccaaagaaacctctgaatttgaaacagggttagtagggacttttatacccagctgggcatcccagaagcctggactctcaggactgtggctagattttgcccatgatctgtagattatgctcttgcaccggagacttgaaagttatgagtttgcattcaaacaaagaaccaccagataaaacagatgttctctaaaactgaggaaaaaaagtttagagatatacactgtatagagaaagaaagctttttgctggattgttctccttgttaaggaaatgtttaaaactagtactcccgggcacctgtgattgcattttataggattctatttagtaatatgatgtctattttacattcagccccaacctacgtcactgaaatagaataggaaatagcagccactatctgagagtacccagttctaggaaagtttggtgcctcctcaagaagtcactatttccatagtcctcaatcatgaatagggcttgtttttgtgataatgtaactattaaacagcaagaaatgcctataacttcagagccttctcatttctatatcttttatcctcttcccagggctttctgatttaaggcaataatgctacactataagtagccttttgtgaaaataccttaattgaggtcacttaagattagatttcagtctgaaagtctacagtttacggagcaaaaggtggagcctaaagaaaccactggcaggtgttttagtcagtggtgtggaaagataatgtttcttgtttcaacccagggcatttttacccatcatgcagtgaggagaaaatacatagttctgaaaaagaacccacactaggtagccctaattttctatctcttcactctaaaaaggatggaaacaagccctactgttccataaccattcccagggatcggctaaggtacattgctgactgctatagactcagtgttcaaggagaaaaaaatcttcagagacttagaaaactctttgcaatattttggtcaggctgatcgtcttgatactcagtgctagaaatgatgctttggattagtagtttccacattctgaatttataggaacactgagtcaccacagccttttttcttgtaaaggtttaagtgatatcagaaatagcaactctacacggaaagcccttgggaatatgaaaatactctctctcaagagcaagggctcttccgtgccccttttctgcctctgtatgtagcctgagcaccagggtagagattgcttttgaaagtttgccccatgtaatctatttcctggctacctaagagaacagccgttttcttcatgaaaacacaaagaggggaaagaggctgctgctgttccagtgggaagttatgtctagccccagaaggcctggtggctgggtcagctcaagcactctcttcatgcactgcaggctcaggaggcattgggttgctttgctttttctatggaattagggagcctattgaaattctagtgcacccctccttttgtttgtcaccaagtcacatggttctgtcttcagtatcctatttttctttttttttaatttctttttctgaggaacaaaattggccatttaaataaagttcttttctagtgagtaaagaggtttctcagagccagaaatcactgaaaagagagtctgtcgaccctgcccatggaaaagcccagagatttctctaaccacttcttgccaaacttcctagttttgtgattggatgtttcttggtttagcattgtttggtgctgaatacattttgcaattcttttgttctctgccctagagcttccattaccctggacttcaactcattaccaaattaaagaattcttttagaagatttcttttaagagtcaggtcacaacagaaagggcgccctcctgttctcctaaatctcaagggcatctcaggttgtgtctgctcttacgttgcaccttccttttgttcccttttaatgcagcagcacactggctatagcagaggcagacctgatttgattatctgataccttttccacaaaatcatatatcccctgctcccagccccaactaatcaaataacatcttctagaacaacagaggaaagctccagaatgggtgtatatcctgtgactcctggccagatccaccttgctccctgtcttcctaggggtcacaggtgttgggagcattgtggaggagccccaacaaggaagcaacatatggctttattatgttttctcaggaatcgaaggggttttataaggggcatatctcatttttgacttctgtgctgagagaaaatattgagttttgggcgcaggcagagcacagacaggacagctggtgttcctgtgtgagggaagtacacatagctcaaggctttaggactgaatgtgaaacaaacatacctggaggaaaacttttttcattatcagaattcacaaattcttactgttcatgggttgaaaaagagtatttgggaccttatagaatattttgatgatacaaaataaaacccttatgacttttaaacacagcaaacccaagtctttctaaggccaagagctactatgatctctaagatgactaggaatgaactgaggctagaatatgagcaggaaattatccagcacacttaatcatggcacaaatagattcaaagcattaggaatttgggaagagaacggtctataaaactgttattaggagctaaagtttacctctcaattaaaagatacaggaaaccattttgatacagagattttcatttcagattttttttctttgcttagcttgtttccccctgtgtagaattgtaacagatccatgtgttccaattattttcttttttaggattatatttcacacatttgggggccttttttgtacaaatattggcatgtaataaggaaaaattgcccatgatgctgagataataccagtgtttttagtggtagaaaatattatttttttataaaccatatctaaatatcttgagataaaaattcccctttgactttttttcctctcccttgtttggcaaattccattttaaaattataaattgctaaaaaatgtcctttccatactatttctctcttccttgtactcatcctaagaagtcttaaatctggaacatttgcttttatcttatctatctgtttcctggctactagaaagaaatttttttagcactcatatcaccctaccatgaaggtctaaatgtaagatgactgtaggacttgaaacaaaaaaaaattaaaaagatccacactcattctttgattttgaagcaaatgtctttccctatttctaaagatatttgtgattgtttaacttaaaagtgagaattgacaatctaaaagcatctctatccttttgaaacaggtccagattggtttatttcctaaaatgtgggtcagtttggaaagtggccatttgatgggccaggaacatagcaataaacaactacctctttgctcctccagattagatctcccactccaatccagcttcttcctctttccacaaaataatttgtcaactattttagaatgtgacatatttgggaaggataaatgtacagtaggaatatgtctactgctatgcaaacctggctggtccattttgtcatggactacaatgattatatcacctcattaagaattctttagggatcctccacctcctcccccactcccttttttttaagagacacttcctttacagggaaaggatgatagactcctcagggtttcaagtcacctgcagctttttctctacatgttctaccaaaagaaaaggtggattctaacccaattgcttagcattttacatggcaaatcagcattaaggcaaatgggtctctctcagatttgagaaacagaaagctacacgtggcccataatggcacctaagatcaacttttcaggcggtattagtgaaaattcttcctactttgctaaatttgaacaaagacactttcaaatctactgtgaaacagtttaaaatattttaaagtggcttttggccttctttcatttgtaacatgtattgagtgatttcatgtcattgtctcctagctttaagagtttttttcttaaggtcaatcttctcttttcattttatgggtggaatcacttgttttccaaaatatcaaaacaattccatgacatagttaattaatgctccctctattggtggtaagtggaaatattagtcttacaacactgctattttaaaaagcaaaattagcaatagaaaaatgaacttactttatctcggaagctgttcctcactaactgttaaaacagatcagttttggacatacagttcttggcaggactcctcttagaaatcacaataggttacacttaatagtcagttaaccacccaagtttacattaaaacttctagcaaaatatccactgaattaagcactgtgggaccaaatcaaactcacaaacacttcagttacactaaccttacaaagcatcacaaagaacttatgaaaaagatccaagttaaccaaatgtctaaaatatatgaataaaaccaatttagtcattacagagttgtttgtgttggaagattttccctcgtttgctgcacagtttttgtaaataaaatgctgacaggaaaattagaaggaaaattaaattaaaatgtaatgtaattttgaaactaaaatacgctctcctttcttctttttaaaactgtagtttggtgttttgctttgtttaaagatttgctttcccctaagtatgttaaaatatgcccagcaatgaaatcactttgggagtttcagctaggtttaagaattcctatatttgagctggaatcccttcaggacactgtctataatgaaaatgtctctattataacaccttgatcaggaccgaggagagaaatccctactaggaagagagagtggcatctggtatgatgcaatagattggtggtcttttgaatggtggctgttggcatctgggaatttttttgttaatttccctaaaacctttcgaagaagcaagggttaattcgtcatctaaagaatgatcatcttattcagccctcttaaccatggtggaaacagtcagaaggtgatatttggaaggaaaaaagtaattttggcatcaatgcatcttgatctataacaggcttctcataatgatgctctttgtagttgggaagggtgaggagctatggcagagttttgtgaactcctcttcctggctgatcacaaaagaaaagaccccatttatcaagacttctagactattagtgtttcactaagaaaaaaagtaaagtcaatagaaattctagaattgtaagatctcaatgaaattttggagaagcaagcaatctctttctgaaagataaagtctcttccatgaaaaagaacagaattctagatgaatcagttgaaaaaattattcagtggggcaacttaagcttgctaaagtcaaagaactacatatcaaaatacaaagcagcaattcaaattacagcagggatgggctggccacagaggccctcatcaacccaggcaatacttaaaataataaaaattaagaaaaattaaaaaaaatatgaagaaaatatccttcctctctttcaaatataactttagttgccttttattctttctatctggaagcagtatcgctaaccttaacagtcttgacttaccaaaaaatatatatatgtgtgtgaaataaaataaaagagaaggaattggtggcagtgtatgcaaaaccaaaatgaaaaaaattacttttaacaatttcactttttttgtttttttttttacacaaatactgttgtaaatatattaaaaaaatcagcattctatctggtaaacgtcacttttgcccctctataaaattttgaattaaaaaagcctcaagaactttttattgttccccccaccctccatttctttttctttttctcttccacaagaatatatcctgacactttttttttttttgcaaagattgttggaaataatccttctcttgtacctagaaacataggtgcaaatttctgatatctttgttttatctgcattcctgcctttcatgaaagtccctcttgattgtgctgaggctgtggctcagcgaagacactgaataaatacgatagccactgttgcttgttgcttgtccaagtcttcctggcttctgctgcaagagggggatatggagaaggtgggccagggtgtgtggacccgggcagaatctggggaagaagcctgccattcgtctttctttcccacaccaccgaacccactgcccttcccacccccacagcccttttatgaaatcagacaacgtggtaggtggaaaacagcagggcctttcctctgggttttcaaccagaagtgatattccacagttttaactggttactgtgaagtccaagcggccagaattgtgaaaatgtccactgaaacactgcaagcggtgtacttaaagacagtaggccttttagattttgttatatattttttgtagtgctcttcacaagtggaaattttttttttttttttacttttttttaaaagatttttttgtaaagaagggttgtatttagaggccagtagctagagatccaaccagtggacctcttgaagcactaccaggccttaaggccaccatccgagggagactgggaaaactattattcacccaagcctccggaaatgtaatgtaccagcaggcaaaaaacagttcttcatgtagtacaaaatgaaacgaaacaaaaacaaaaacagaaagtaaaaatgaaaccaaaacatttcttaaattctagtgccatagcttttttgtttgtttgttttttgttgttgttttgttttgttcataagaaagagagaaagatactacttatccgtcagacacatgcatcctcatgtggtcgttgaactgctcgatttggtcaaactttgctgggcagacggagcagacgtaagtggtcccctccgtgcaggccaccacgcctggggggccagcgcgggcacctgggggtgtgcctgcagggggggtcccattgctggcactgtgcagggccacgtgtcgctccaggagggtcttgtgagagaacttctttttgcagatgtagcactcgtaggacttctctccccggtggaggcgcatgtgcacgttgagggagctcttctgggtgaagcgcttgttgcagatactacactggtatgccctcactcctgtgtgtgtcaccatgtgcttgataaggtaatcctttaaggagaaggagcgccaacagatgctgcattggtggggcttctcacctgtgtgtacgaacatgtgcttgacgtagttctgtttggcggtgaaagtcttgttgcagagagtgcactcataaggctttttttcgccttgcccactggctgtgctgtggcctgcggatgaggccaggggctgtggcgctggcagctgtgcagtaaaggtcgacagaccgggctgggacactgtcacaaactgggtctgctggcctgccaggggctgtggcaggctgaagaggaaaggcttggggccactgcccgcgggctgggtagtgaagagggctggcaggtaggtgttgccagctgtgccaatgacctgcgtgttgctggtcaaggtcagaggcatcctcaggttgctggtgagggtttctgtctggcgtaagtagagctgggtacttggcaatggctgcccgatggacgtgttgaccgaaggctgttgtaggacgctcttgtcggagctgttgctgacagtgataacagtgctgtccatctccacttcattgcttctctccggagaggaagcacctgtttctagctggtttgtctgcggaccaccctcagcgggggcttctgcagcctgctcgggttgggtgggttcagcctggctgtcccgcgccgccccaggcccaaactgctgctccaccgagtcaggctcggtgcctatggaggagctgacgcccgagtcgaagctttcacctttgggctcactctcggtgccctcggcctggtctgtgtcttccgtgcactcctcggattcgttgcgttccaggatctgcaccctttgctgcccgtagtagtcgtaatcgtcctccatctcctgcttgatgtggatgttgcccactagggtctggatgcgcacaggccggggctgcttgcggcagtgcgtggtctcgggggtggtggacaggtagcgctccatctgctgcgagcgctcatggatgcgtgtgatccagctggggtcttccatgtggtggtcgcggggcaggccgagcgcagtctcgtggtggctgaccactgcgccgctgtaaaaagagcgctcgccgctgccattctgcatggagcacgcgtagagtgccgagtagatcctgtccacgctgtgctgtgggtggctctgcaggtagcccgactccgtgtcgctgctctggcctgacgtgcctgactcgggagtgccccgcggcgtgtcctggcccgagtcctggatccccgggaacacatcgcccacgttctgtgacacgatgcgcgtgcactcgtcgatgactgttttgatctgcaggatgctggcggccgtgaggatctgcagagcttccgactgcgagacccgtagcacgccgctgtacatgaagtcaatgagcttttgcactgactgcactgacaccaccgacgggatctcgatgtcgctgtagccaagcagcagtttgtcctggaagaaggggctgccggctgccagcacgcagcggtgtgcgcgcagcatgctcccgtggatgcgcaccgttacgtcacagaagtggccacggttgcgctgctcgttgagggtctcgagcacggaattgctgaagttgtgaaggttgatgctgtgaatgcgctcggtcatccccttgcaactgatgtcacaatcagatgacccggtgtgagcgtgagagtttgtcagtgaatgtgttgagtggatgagggctgggtctggagacaaaacagcttcaaagttcaggcagggaaggcccggcttggcgctggatccacccggctgagtaatctcattctcctcagatgccttctggttttcagctgtcttgggtttcttcagtagtttcaaaatcaatggtgtcactcttcaggtaaattactccaaggcttgggcctagtgcagatgttcattggggcagggagcagagagcggctgcatgtaaagagaaggggcaggtcacagactgatggtcaaagatcagacagcaatgtcatgaggaatatcctgttagtaatgatgaaacattaggaatacagtgcagctcaatcttttgtttttaaggtgcagtgatttcagtctctaaatgtaacttcaggcagtctgtgcagctatggggcacaaacttgcaattcatcaattcttcagccttcagagtcccaaaggcaattcttaacacttctttttatttgtcgtgaaagggcatattgctgtggaggctggtaggcagcaaacttgtcacctgatcttcatatgcacaaggcctgtattccactggtctataaaatctcctcgcgctctttaatcttctttcctcaactcctaaacttccccccgcccctacttcttcggcagaag

SEQ ID NO: 16683 - RNA, 12673 nt, Homo sapiens
  source 1..12673: mol_type = other RNA
taaaacccacaattatgtttgtctagtagaaatatatctgctggaacactttggagaacagattggtaattttgccattacactagacattagccctttcaaagcagactaagagtacgtagttccttagtgaatacaaggcttcacaactgaagagcattgcagggagcttggctaaggtgaaaagggacttgctggagaggtacagcagaatgggatgggattagaaaacaacaatctattaggaaagatgaaaggaaggaattccccagtgttcacgctgagaagtcttcatattggaccagtgtgagggggtcttttatactgaggttttaaaaacctgacttcattttgtcctgaatgtagaagtgaagaaggacactagtttcaggcacctgggatggtggaaaagtttattcaactgaggctttccatgcattgggttgaatagctgagggaagctgaagactcttatctgaaaatatgatctgaaaatatttattgtataggaagacagaatgcctgatttctgaagttttcttgatggcccaactaaagaagaaaggcaccaaatcctcactttaacaggtaaatggagatcctgagggctggatacccaagagccaccattttacggattcctcagatttaaaaatgtctcagatagatatttccaaattctatttctattagcctctgtggataaagagttcctgaaactctggttttactttttttggaaaaaaaaaaaaaaaaaaaaaaaaaaaacaactcccaggaaaatgaacactatattgccaagctgcctccagggaaaggttgaagactagttaaaataattctaagcgtattgaaaaaagaaagtgtaaagatccagtattaaaatgaatgtttgagaatacagtggggacaactaggtaattcactgtcttacgcttttcagaagactggccctttgaaacgcagcctgttattgttggtcagatcatgtggcacttaagtagccccttggtcatatttttaaaagcaaatatagacagtgacagtcctacaggggaaaatcacagatacattcatatgcacctcttttgttcttcagatattgagtgggtcagctaaacaagatcactttgaatatgaacctctttgtattagtcacaccaacaaaaaagtttcaaaaaaagttttcactttcctacatttgctaagtctgagctttaaaaaattctaaaatcctctaaagacaatactgaagctgataatataaaaagcaaattagagcactaatgattattactagatgcaccagattaactgcagcaggttggtgatgggtgatataagcaaagacataatatttcaatcaactcatgatcataggcagattcaaaagttaaaatgaatataatgtaatatatatttcaatatagagttgttatatataatgtgtatgtcctaggtttcagaaatactgcaatgtagtgtattgtagttaagtaagcatacctaaatagtaactcatattctttcacaaagtcactagtactgttaattaaaggaaaaaataaaaccgaaacaactaattgtttttccagtaaaaagaaatacctatggttacagttacagacttcttttggatatagaaagacaatatacattttaaaaagtaataacgacaaaaaagttgcaactgtaagtagccttacttaacaggggaaggggaaaagtcaccagaatagaagaggaaagaaaatgtcctctgacttctgtaaaacagaaataatgtacaaatcataaaaaataacaaaccatctagtaaaagaagggcatgggagtgagaaaactgaatcctgaattccaggccaccaaaccctcagagtccattcattcagtatattatactagagtggcattctacttcaatgcttgagatgggcaagagcaatcaattcctacagattaccaaaaaacattccccccaacagtctattggtttgctagacatggtaaacaacccactcctggaaagactttggcaaaggccacattggtttcaggagacacagtttgtgaattacgatgatatcttgtgagtacaggcagaattaggaagctttagtttgagaataaaatttatgtgtgtgtgtgtgtgtgtgtgtgtgtgtgtgcacactgcattgcatagaggaaaggaatgaagacctttgagctatgggatggctcaggccaaagtttgtgtgggctttgcctgcctggcattggtccccacccctgccacctccaggagacctggggagacgccctggactgctgctccctcttgtctgctcaccagttgaagacttctgttataccttattatggaggaaaacagcctgtccctgtgggtttgctgtggattcaacaagctgcatttgtttctcccaattctgaaacattacaaaaagcaacagagtgggcaggtgactgcttcctgggaagggagccacaagtcttaaacacaatggtgggaagaggcaactgtatctatgcacgaggacctctgcctgtgtgtgcttcctttggggggcacacacacttccagatgacaataagtatatacacaaacacacacatgtgcacacatgtcaataaatccaatagaactgtagagtttgttaaatgcactctactccacataagcatattcaagtttctcatgaaacggatacatagaaattactgatggttgggctccttcagaatgccctaaagtctcatcacagatactgatgcacccaactaaggcaacaaagcataagcagatacgtgagatatgtcagaccttcgacttctaaccagaagttcaaaaatgtatcttgttgtcactgggcaatatgaatgtgaaacagttttgtgctgagggaagctcacactgtgtgtgcacatgtataaataatgtatactcatttatagacattttggacagcagcggtgacatactggatgggttaagactctttcattattagaatctacatataaattgcaatgagtttgctgggtaaaaacaactgttgcaacactagtagaaacagatgcccccaaggtttttttttttttttttttttttttctctcttggatgtatcaaaatctcattgaggcattctaaaccaaagaaacctctgaatttgaaacagggttagtagggacttttatacccagctgggcatcccagaagcctggactctcaggactgtggctagattttgcccatgatctgtagattatgctcttgcaccggagacttgaaagttatgagtttgcattcaaacaaagaaccaccagataaaacagatgttctctaaaactgaggaaaaaaagtttagagatatacactgtatagagaaagaaagctttttgctggattgttctccttgttaaggaaatgtttaaaactagtactcccgggcacctgtgattgcattttataggattctatttagtaatatgatgtctattttacattcagccccaacctacgtcactgaaatagaataggaaatagcagccactatctgagagtacccagttctaggaaagtttggtgcctcctcaagaagtcactatttccatagtcctcaatcatgaatagggcttgtttttgtgataatgtaactattaaacagcaagaaatgcctataacttcagagccttctcatttctatatcttttatcctcttcccagggctttctgatttaaggcaataatgctacactataagtagccttttgtgaaaataccttaattgaggtcacttaagattagatttcagtctgaaagtctacagtttacggagcaaaaggtggagcctaaagaaaccactggcaggtgttttagtcagtggtgtggaaagataatgtttcttgtttcaacccagggcatttttacccatcatgcagtgaggagaaaatacatagttctgaaaaagaacccacactaggtagccctaattttctatctcttcactctaaaaaggatggaaacaagccctactgttccataaccattcccagggatcggctaaggtacattgctgactgctatagactcagtgttcaaggagaaaaaaatcttcagagacttagaaaactctttgcaatattttggtcaggctgatcgtcttgatactcagtgctagaaatgatgctttggattagtagtttccacattctgaatttataggaacactgagtcaccacagccttttttcttgtaaaggtttaagtgatatcagaaatagcaactctacacggaaagcccttgggaatatgaaaatactctctctcaagagcaagggctcttccgtgccccttttctgcctctgtatgtagcctgagcaccagggtagagattgcttttgaaagtttgccccatgtaatctatttcctggctacctaagagaacagccgttttcttcatgaaaacacaaagaggggaaagaggctgctgctgttccagtgggaagttatgtctagccccagaaggcctggtggctgggtcagctcaagcactctcttcatgcactgcaggctcaggaggcattgggttgctttgctttttctatggaattagggagcctattgaaattctagtgcacccctccttttgtttgtcaccaagtcacatggttctgtcttcagtatcctatttttctttttttttaatttctttttctgaggaacaaaattggccatttaaataaagttcttttctagtgagtaaagaggtttctcagagccagaaatcactgaaaagagagtctgtcgaccctgcccatggaaaagcccagagatttctctaaccacttcttgccaaacttcctagttttgtgattggatgtttcttggtttagcattgtttggtgctgaatacattttgcaattcttttgttctctgccctagagcttccattaccctggacttcaactcattaccaaattaaagaattcttttagaagatttcttttaagagtcaggtcacaacagaaagggcgccctcctgttctcctaaatctcaagggcatctcaggttgtgtctgctcttacgttgcaccttccttttgttcccttttaatgcagcagcacactggctatagcagaggcagacctgatttgattatctgataccttttccacaaaatcatatatcccctgctcccagccccaactaatcaaataacatcttctagaacaacagaggaaagctccagaatgggtgtatatcctgtgactcctggccagatccaccttgctccctgtcttcctaggggtcacaggtgttgggagcattgtggaggagccccaacaaggaagcaacatatggctttattatgttttctcaggaatcgaaggggttttataaggggcatatctcatttttgacttctgtgctgagagaaaatattgagttttgggcgcaggcagagcacagacaggacagctggtgttcctgtgtgagggaagtacacatagctcaaggctttaggactgaatgtgaaacaaacatacctggaggaaaacttttttcattatcagaattcacaaattcttactgttcatgggttgaaaaagagtatttgggaccttatagaatattttgatgatacaaaataaaacccttatgacttttaaacacagcaaacccaagtctttctaaggccaagagctactatgatctctaagatgactaggaatgaactgaggctagaatatgagcaggaaattatccagcacacttaatcatggcacaaatagattcaaagcattaggaatttgggaagagaacggtctataaaactgttattaggagctaaagtttacctctcaattaaaagatacaggaaaccattttgatacagagattttcatttcagattttttttctttgcttagcttgtttccccctgtgtagaattgtaacagatccatgtgttccaattattttcttttttaggattatatttcacacatttgggggccttttttgtacaaatattggcatgtaataaggaaaaattgcccatgatgctgagataataccagtgtttttagtggtagaaaatattatttttttataaaccatatctaaatatcttgagataaaaattcccctttgactttttttcctctcccttgtttggcaaattccattttaaaattataaattgctaaaaaatgtcctttccatactatttctctcttccttgtactcatcctaagaagtcttaaatctggaacatttgcttttatcttatctatctgtttcctggctactagaaagaaatttttttagcactcatatcaccctaccatgaaggtctaaatgtaagatgactgtaggacttgaaacaaaaaaaaattaaaaagatccacactcattctttgattttgaagcaaatgtctttccctatttctaaagatatttgtgattgtttaacttaaaagtgagaattgacaatctaaaagcatctctatccttttgaaacaggtccagattggtttatttcctaaaatgtgggtcagtttggaaagtggccatttgatgggccaggaacatagcaataaacaactacctctttgctcctccagattagatctcccactccaatccagcttcttcctctttccacaaaataatttgtcaactattttagaatgtgacatatttgggaaggataaatgtacagtaggaatatgtctactgctatgcaaacctggctggtccattttgtcatggactacaatgattatatcacctcattaagaattctttagggatcctccacctcctcccccactcccttttttttaagagacacttcctttacagggaaaggatgatagactcctcagggtttcaagtcacctgcagctttttctctacatgttctaccaaaagaaaaggtggattctaacccaattgcttagcattttacatggcaaatcagcattaaggcaaatgggtctctctcagatttgagaaacagaaagctacacgtggcccataatggcacctaagatcaacttttcaggcggtattagtgaaaattcttcctactttgctaaatttgaacaaagacactttcaaatctactgtgaaacagtttaaaatattttaaagtggcttttggccttctttcatttgtaacatgtattgagtgatttcatgtcattgtctcctagctttaagagtttttttcttaaggtcaatcttctcttttcattttatgggtggaatcacttgttttccaaaatatcaaaacaattccatgacatagttaattaatgctccctctattggtggtaagtggaaatattagtcttacaacactgctattttaaaaagcaaaattagcaatagaaaaatgaacttactttatctcggaagctgttcctcactaactgttaaaacagatcagttttggacatacagttcttggcaggactcctcttagaaatcacaataggttacacttaatagtcagttaaccacccaagtttacattaaaacttctagcaaaatatccactgaattaagcactgtgggaccaaatcaaactcacaaacacttcagttacactaaccttacaaagcatcacaaagaacttatgaaaaagatccaagttaaccaaatgtctaaaatatatgaataaaaccaatttagtcattacagagttgtttgtgttggaagattttccctcgtttgctgcacagtttttgtaaataaaatgctgacaggaaaattagaaggaaaattaaattaaaatgtaatgtaattttgaaactaaaatacgctctcctttcttctttttaaaactgtagtttggtgttttgctttgtttaaagatttgctttcccctaagtatgttaaaatatgcccagcaatgaaatcactttgggagtttcagctaggtttaagaattcctatatttgagctggaatcccttcaggacactgtctataatgaaaatgtctctattataacaccttgatcaggaccgaggagagaaatccctactaggaagagagagtggcatctggtatgatgcaatagattggtggtcttttgaatggtggctgttggcatctgggaatttttttgttaatttccctaaaacctttcgaagaagcaagggttaattcgtcatctaaagaatgatcatcttattcagccctcttaaccatggtggaaacagtcagaaggtgatatttggaaggaaaaaagtaattttggcatcaatgcatcttgatctataacaggcttctcataatgatgctctttgtagttgggaagggtgaggagctatggcagagttttgtgaactcctcttcctggctgatcacaaaagaaaagaccccatttatcaagacttctagactattagtgtttcactaagaaaaaaagtaaagtcaatagaaattctagaattgtaagatctcaatgaaattttggagaagcaagcaatctctttctgaaagataaagtctcttccatgaaaaagaacagaattctagatgaatcagttgaaaaaattattcagtggggcaacttaagcttgctaaagtcaaagaactacatatcaaaatacaaagcagcaattcaaattacagcagggatgggctggccacagaggccctcatcaacccaggcaatacttaaaataataaaaattaagaaaaattaaaaaaaatatgaagaaaatatccttcctctctttcaaatataactttagttgccttttattctttctatctggaagcagtatcgctaaccttaacagtcttgacttaccaaaaaatatatatatgtgtgtgaaataaaataaaagagaaggaattggtggcagtgtatgcaaaaccaaaatgaaaaaaattacttttaacaatttcactttttttgtttttttttttacacaaatactgttgtaaatatattaaaaaaatcagcattctatctggtaaacgtcacttttgcccctctataaaattttgaattaaaaaagcctcaagaactttttattgttccccccaccctccatttctttttctttttctcttccacaagaatatatcctgacactttttttttttttgcaaagattgttggaaataatccttctcttgtacctagaaacataggtgcaaatttctgatatctttgttttatctgcattcctgcctttcatgaaagtccctcttgattgtgctgaggctgtggctcagcgaagacactgaataaatacgatagccactgttgcttgttgcttgtccaagtcttcctggcttctgctgcaagagggggatatggagaaggtgggccagggtgtgtggacccgggcagaatctggggaagaagcctgccattcgtctttctttcccacaccaccgaacccactgcccttcccacccccacagcccttttatgaaatcagacaacgtggtaggtggaaaacagcagggcctttcctctgggttttcaaccagaagtgatattccacagttttaactggttactgtgaagtccaagcggccagaattgtgaaaatgtccactgaaacactgcaagcggtgtacttaaagacagtaggccttttagattttgttatatattttttgtagtgctcttcacaagtggaaattttttttttttttttacttttttttaaaagatttttttgtaaagaagggttgtatttagaggccagtagctagagatccaaccagtggacctcttgaagcactaccaggccttaaggccaccatccgagggagactgggaaaactattattcacccaagcctccggaaatgtaatgtaccagcaggcaaaaaacagttcttcatgtagtacaaaatgaaacgaaacaaaaacaaaaacagaaagtaaaaatgaaaccaaaacatttcttaaattctagtgccatagcttttttgtttgtttgttttttgttgttgttttgttttgttcataagaaagagagaaagatactacttatccgtcagacacatgcatcctcatgtggtcgttgaactgctcgatttggtcaaactttgctgggcagacggagcagacgtaagtggtcccctccgtgcaggccaccacgcctggggggccagcgcgggcacctgggggtgtgcctgcagggggggtcccattgctggcactgtgcagggccacgtgtcgctccaggagggtcttgtgagagaacttctttttgcagatgtagcactcgtaggacttctctccccggtggaggcgcatgtgcacgttgagggagctcttctgggtgaagcgcttgttgcagatactacactggtatgccctcactcctgtgtgtgtcaccatgtgcttgataaggtaatcctttaaggagaaggagcgccaacagatgctgcattggtggggcttctcacctgtgtgtacgaacatgtgcttgacgtagttctgtttggcggtgaaagtcttgttgcagagagtgcactcataaggctttttttcgccttgcccactggctgtgctgtggcctgcggatgaggccaggggctgtggcgctggcagctgtgcagtaaaggtcgacagaccgggctgggacactgtcacaaactgggtctgctggcctgccaggggctgtggcaggctgaagaggaaaggcttggggccactgcccgcgggctgggtagtgaagagggctggcaggtaggtgttgccagctgtgccaatgacctgcgtgttgctggtcaaggtcagaggcatcctcaggttgctggtgagggtttctgtctggcgtaagtagagctgggtacttggcaatggctgcccgatggacgtgttgaccgaaggctgttgtaggacgctcttgtcggagctgttgctgacagtgataacagtgctgtccatctccacttcattgcttctctccggagaggaagcacctgtttctagctggtttgtctgcggaccaccctcagcgggggcttctgcagcctgctcgggttgggtgggttcagcctggctgtcccgcgccgccccaggcccaaactgctgctccaccgagtcaggctcggtgcctatggaggagctgacgcccgagtcgaagctttcacctttgggctcactctcggtgccctcggcctggtctgtgtcttccgtgcactcctcggattcgttgcgttccaggatctgcaccctttgctgcccgtagtagtcgtaatcgtcctccatctcctgcttgatgtggatgttgcccactagggtctggatgcgcacaggccggggctgcttgcggcagtgcgtggtctcgggggtggtggacaggtagcgctccatctgctgcgagcgctcatggatgcgtgtgatccagctggggtcttccatgtggtggtcgcggggcaggccgagcgcagtctcgtggtggctgaccactgcgccgctgtaaaaagagcgctcgccgctgccattctgcatggagcacgcgtagagtgccgagtagatcctgtccacgctgtgctgtgggtggctctgcaggtagcccgactccgtgtcgctgctctggcctgacgtgcctgactcgggagtgccccgcggcgtgtcctggcccgagtcctggatccccgggaacacatcgcccacgttctgtgacacgatgcgcgtgcactcgtcgatgactgttttgatctgcaggatgctggcggccgtgaggatctgcagagcttccgactgcgagacccgtagcacgccgctgtacatgaagtcaatgagcttttgcactgactgcactgacaccaccgacgggatctcgatgtcgctgtagccaagcagcagtttgtcctggaagaaggggctgccggctgccagcacgcagcggtgtgcgcgcagcatgctcccgtggatgcgcaccgttacgtcacagaagtggccacggttgcgctgctcgttgagggtctcgagcacggaattgctgaagttgtgaaggttgatgctgtgaatgcgctcggtcatccccttgcaactgatgtcacaatcagatgacccggtgtgagcgtgagagtttgtcagtgaatgtgttgagtggatgagggctgggtctggagacaaaacagcttcaaagttcaggcagggaaggcccggcttggcgctggatccacccggctgagtaatctcattctcctcagatgccttctggttttcagctgtcttgggtttcttcagtagtttcaaaatcaatggtgtcactcttcaggtaaattactccaaggcttgggcctagtgcagatgttcattggggcagggagcagagagcggctgcatgtaaagagaaggggcaggtcacagactgatggtcaaagatcagacagcaatgtcatgaggaatatcctgttagtaatgatgaaacattaggaatacagtgcagctcaatcttttgtttttaaggtgcagtgatttcagtctctaaatgtaacttcaggcagtctgtgcagctatggggcacaaacttgcaattcatcaattcttcagccttcagagtcccaaaggcaattcttaacacttctttttatttgtctcctcgcgctctttaatcttctttcctcaactcctaaacttccccccgcccctacttcttcggcagaag

SEQ ID NO: 16684 - RNA, 12737 nt, Homo sapiens
  source 1..12737: mol_type = other RNA
taaaacccacaattatgtttgtctagtagaaatatatctgctggaacactttggagaacagattggtaattttgccattacactagacattagccctttcaaagcagactaagagtacgtagttccttagtgaatacaaggcttcacaactgaagagcattgcagggagcttggctaaggtgaaaagggacttgctggagaggtacagcagaatgggatgggattagaaaacaacaatctattaggaaagatgaaaggaaggaattccccagtgttcacgctgagaagtcttcatattggaccagtgtgagggggtcttttatactgaggttttaaaaacctgacttcattttgtcctgaatgtagaagtgaagaaggacactagtttcaggcacctgggatggtggaaaagtttattcaactgaggctttccatgcattgggttgaatagctgagggaagctgaagactcttatctgaaaatatgatctgaaaatatttattgtataggaagacagaatgcctgatttctgaagttttcttgatggcccaactaaagaagaaaggcaccaaatcctcactttaacaggtaaatggagatcctgagggctggatacccaagagccaccattttacggattcctcagatttaaaaatgtctcagatagatatttccaaattctatttctattagcctctgtggataaagagttcctgaaactctggttttactttttttggaaaaaaaaaaaaaaaaaaaaaaaaaaaacaactcccaggaaaatgaacactatattgccaagctgcctccagggaaaggttgaagactagttaaaataattctaagcgtattgaaaaaagaaagtgtaaagatccagtattaaaatgaatgtttgagaatacagtggggacaactaggtaattcactgtcttacgcttttcagaagactggccctttgaaacgcagcctgttattgttggtcagatcatgtggcacttaagtagccccttggtcatatttttaaaagcaaatatagacagtgacagtcctacaggggaaaatcacagatacattcatatgcacctcttttgttcttcagatattgagtgggtcagctaaacaagatcactttgaatatgaacctctttgtattagtcacaccaacaaaaaagtttcaaaaaaagttttcactttcctacatttgctaagtctgagctttaaaaaattctaaaatcctctaaagacaatactgaagctgataatataaaaagcaaattagagcactaatgattattactagatgcaccagattaactgcagcaggttggtgatgggtgatataagcaaagacataatatttcaatcaactcatgatcataggcagattcaaaagttaaaatgaatataatgtaatatatatttcaatatagagttgttatatataatgtgtatgtcctaggtttcagaaatactgcaatgtagtgtattgtagttaagtaagcatacctaaatagtaactcatattctttcacaaagtcactagtactgttaattaaaggaaaaaataaaaccgaaacaactaattgtttttccagtaaaaagaaatacctatggttacagttacagacttcttttggatatagaaagacaatatacattttaaaaagtaataacgacaaaaaagttgcaactgtaagtagccttacttaacaggggaaggggaaaagtcaccagaatagaagaggaaagaaaatgtcctctgacttctgtaaaacagaaataatgtacaaatcataaaaaataacaaaccatctagtaaaagaagggcatgggagtgagaaaactgaatcctgaattccaggccaccaaaccctcagagtccattcattcagtatattatactagagtggcattctacttcaatgcttgagatgggcaagagcaatcaattcctacagattaccaaaaaacattccccccaacagtctattggtttgctagacatggtaaacaacccactcctggaaagactttggcaaaggccacattggtttcaggagacacagtttgtgaattacgatgatatcttgtgagtacaggcagaattaggaagctttagtttgagaataaaatttatgtgtgtgtgtgtgtgtgtgtgtgtgtgtgtgcacactgcattgcatagaggaaaggaatgaagacctttgagctatgggatggctcaggccaaagtttgtgtgggctttgcctgcctggcattggtccccacccctgccacctccaggagacctggggagacgccctggactgctgctccctcttgtctgctcaccagttgaagacttctgttataccttattatggaggaaaacagcctgtccctgtgggtttgctgtggattcaacaagctgcatttgtttctcccaattctgaaacattacaaaaagcaacagagtgggcaggtgactgcttcctgggaagggagccacaagtcttaaacacaatggtgggaagaggcaactgtatctatgcacgaggacctctgcctgtgtgtgcttcctttggggggcacacacacttccagatgacaataagtatatacacaaacacacacatgtgcacacatgtcaataaatccaatagaactgtagagtttgttaaatgcactctactccacataagcatattcaagtttctcatgaaacggatacatagaaattactgatggttgggctccttcagaatgccctaaagtctcatcacagatactgatgcacccaactaaggcaacaaagcataagcagatacgtgagatatgtcagaccttcgacttctaaccagaagttcaaaaatgtatcttgttgtcactgggcaatatgaatgtgaaacagttttgtgctgagggaagctcacactgtgtgtgcacatgtataaataatgtatactcatttatagacattttggacagcagcggtgacatactggatgggttaagactctttcattattagaatctacatataaattgcaatgagtttgctgggtaaaaacaactgttgcaacactagtagaaacagatgcccccaaggtttttttttttttttttttttttttctctcttggatgtatcaaaatctcattgaggcattctaaaccaaagaaacctctgaatttgaaacagggttagtagggacttttatacccagctgggcatcccagaagcctggactctcaggactgtggctagattttgcccatgatctgtagattatgctcttgcaccggagacttgaaagttatgagtttgcattcaaacaaagaaccaccagataaaacagatgttctctaaaactgaggaaaaaaagtttagagatatacactgtatagagaaagaaagctttttgctggattgttctccttgttaaggaaatgtttaaaactagtactcccgggcacctgtgattgcattttataggattctatttagtaatatgatgtctattttacattcagccccaacctacgtcactgaaatagaataggaaatagcagccactatctgagagtacccagttctaggaaagtttggtgcctcctcaagaagtcactatttccatagtcctcaatcatgaatagggcttgtttttgtgataatgtaactattaaacagcaagaaatgcctataacttcagagccttctcatttctatatcttttatcctcttcccagggctttctgatttaaggcaataatgctacactataagtagccttttgtgaaaataccttaattgaggtcacttaagattagatttcagtctgaaagtctacagtttacggagcaaaaggtggagcctaaagaaaccactggcaggtgttttagtcagtggtgtggaaagataatgtttcttgtttcaacccagggcatttttacccatcatgcagtgaggagaaaatacatagttctgaaaaagaacccacactaggtagccctaattttctatctcttcactctaaaaaggatggaaacaagccctactgttccataaccattcccagggatcggctaaggtacattgctgactgctatagactcagtgttcaaggagaaaaaaatcttcagagacttagaaaactctttgcaatattttggtcaggctgatcgtcttgatactcagtgctagaaatgatgctttggattagtagtttccacattctgaatttataggaacactgagtcaccacagccttttttcttgtaaaggtttaagtgatatcagaaatagcaactctacacggaaagcccttgggaatatgaaaatactctctctcaagagcaagggctcttccgtgccccttttctgcctctgtatgtagcctgagcaccagggtagagattgcttttgaaagtttgccccatgtaatctatttcctggctacctaagagaacagccgttttcttcatgaaaacacaaagaggggaaagaggctgctgctgttccagtgggaagttatgtctagccccagaaggcctggtggctgggtcagctcaagcactctcttcatgcactgcaggctcaggaggcattgggttgctttgctttttctatggaattagggagcctattgaaattctagtgcacccctccttttgtttgtcaccaagtcacatggttctgtcttcagtatcctatttttctttttttttaatttctttttctgaggaacaaaattggccatttaaataaagttcttttctagtgagtaaagaggtttctcagagccagaaatcactgaaaagagagtctgtcgaccctgcccatggaaaagcccagagatttctctaaccacttcttgccaaacttcctagttttgtgattggatgtttcttggtttagcattgtttggtgctgaatacattttgcaattcttttgttctctgccctagagcttccattaccctggacttcaactcattaccaaattaaagaattcttttagaagatttcttttaagagtcaggtcacaacagaaagggcgccctcctgttctcctaaatctcaagggcatctcaggttgtgtctgctcttacgttgcaccttccttttgttcccttttaatgcagcagcacactggctatagcagaggcagacctgatttgattatctgataccttttccacaaaatcatatatcccctgctcccagccccaactaatcaaataacatcttctagaacaacagaggaaagctccagaatgggtgtatatcctgtgactcctggccagatccaccttgctccctgtcttcctaggggtcacaggtgttgggagcattgtggaggagccccaacaaggaagcaacatatggctttattatgttttctcaggaatcgaaggggttttataaggggcatatctcatttttgacttctgtgctgagagaaaatattgagttttgggcgcaggcagagcacagacaggacagctggtgttcctgtgtgagggaagtacacatagctcaaggctttaggactgaatgtgaaacaaacatacctggaggaaaacttttttcattatcagaattcacaaattcttactgttcatgggttgaaaaagagtatttgggaccttatagaatattttgatgatacaaaataaaacccttatgacttttaaacacagcaaacccaagtctttctaaggccaagagctactatgatctctaagatgactaggaatgaactgaggctagaatatgagcaggaaattatccagcacacttaatcatggcacaaatagattcaaagcattaggaatttgggaagagaacggtctataaaactgttattaggagctaaagtttacctctcaattaaaagatacaggaaaccattttgatacagagattttcatttcagattttttttctttgcttagcttgtttccccctgtgtagaattgtaacagatccatgtgttccaattattttcttttttaggattatatttcacacatttgggggccttttttgtacaaatattggcatgtaataaggaaaaattgcccatgatgctgagataataccagtgtttttagtggtagaaaatattatttttttataaaccatatctaaatatcttgagataaaaattcccctttgactttttttcctctcccttgtttggcaaattccattttaaaattataaattgctaaaaaatgtcctttccatactatttctctcttccttgtactcatcctaagaagtcttaaatctggaacatttgcttttatcttatctatctgtttcctggctactagaaagaaatttttttagcactcatatcaccctaccatgaaggtctaaatgtaagatgactgtaggacttgaaacaaaaaaaaattaaaaagatccacactcattctttgattttgaagcaaatgtctttccctatttctaaagatatttgtgattgtttaacttaaaagtgagaattgacaatctaaaagcatctctatccttttgaaacaggtccagattggtttatttcctaaaatgtgggtcagtttggaaagtggccatttgatgggccaggaacatagcaataaacaactacctctttgctcctccagattagatctcccactccaatccagcttcttcctctttccacaaaataatttgtcaactattttagaatgtgacatatttgggaaggataaatgtacagtaggaatatgtctactgctatgcaaacctggctggtccattttgtcatggactacaatgattatatcacctcattaagaattctttagggatcctccacctcctcccccactcccttttttttaagagacacttcctttacagggaaaggatgatagactcctcagggtttcaagtcacctgcagctttttctctacatgttctaccaaaagaaaaggtggattctaacccaattgcttagcattttacatggcaaatcagcattaaggcaaatgggtctctctcagatttgagaaacagaaagctacacgtggcccataatggcacctaagatcaacttttcaggcggtattagtgaaaattcttcctactttgctaaatttgaacaaagacactttcaaatctactgtgaaacagtttaaaatattttaaagtggcttttggccttctttcatttgtaacatgtattgagtgatttcatgtcattgtctcctagctttaagagtttttttcttaaggtcaatcttctcttttcattttatgggtggaatcacttgttttccaaaatatcaaaacaattccatgacatagttaattaatgctccctctattggtggtaagtggaaatattagtcttacaacactgctattttaaaaagcaaaattagcaatagaaaaatgaacttactttatctcggaagctgttcctcactaactgttaaaacagatcagttttggacatacagttcttggcaggactcctcttagaaatcacaataggttacacttaatagtcagttaaccacccaagtttacattaaaacttctagcaaaatatccactgaattaagcactgtgggaccaaatcaaactcacaaacacttcagttacactaaccttacaaagcatcacaaagaacttatgaaaaagatccaagttaaccaaatgtctaaaatatatgaataaaaccaatttagtcattacagagttgtttgtgttggaagattttccctcgtttgctgcacagtttttgtaaataaaatgctgacaggaaaattagaaggaaaattaaattaaaatgtaatgtaattttgaaactaaaatacgctctcctttcttctttttaaaactgtagtttggtgttttgctttgtttaaagatttgctttcccctaagtatgttaaaatatgcccagcaatgaaatcactttgggagtttcagctaggtttaagaattcctatatttgagctggaatcccttcaggacactgtctataatgaaaatgtctctattataacaccttgatcaggaccgaggagagaaatccctactaggaagagagagtggcatctggtatgatgcaatagattggtggtcttttgaatggtggctgttggcatctgggaatttttttgttaatttccctaaaacctttcgaagaagcaagggttaattcgtcatctaaagaatgatcatcttattcagccctcttaaccatggtggaaacagtcagaaggtgatatttggaaggaaaaaagtaattttggcatcaatgcatcttgatctataacaggcttctcataatgatgctctttgtagttgggaagggtgaggagctatggcagagttttgtgaactcctcttcctggctgatcacaaaagaaaagaccccatttatcaagacttctagactattagtgtttcactaagaaaaaaagtaaagtcaatagaaattctagaattgtaagatctcaatgaaattttggagaagcaagcaatctctttctgaaagataaagtctcttccatgaaaaagaacagaattctagatgaatcagttgaaaaaattattcagtggggcaacttaagcttgctaaagtcaaagaactacatatcaaaatacaaagcagcaattcaaattacagcagggatgggctggccacagaggccctcatcaacccaggcaatacttaaaataataaaaattaagaaaaattaaaaaaaatatgaagaaaatatccttcctctctttcaaatataactttagttgccttttattctttctatctggaagcagtatcgctaaccttaacagtcttgacttaccaaaaaatatatatatgtgtgtgaaataaaataaaagagaaggaattggtggcagtgtatgcaaaaccaaaatgaaaaaaattacttttaacaatttcactttttttgtttttttttttacacaaatactgttgtaaatatattaaaaaaatcagcattctatctggtaaacgtcacttttgcccctctataaaattttgaattaaaaaagcctcaagaactttttattgttccccccaccctccatttctttttctttttctcttccacaagaatatatcctgacactttttttttttttgcaaagattgttggaaataatccttctcttgtacctagaaacataggtgcaaatttctgatatctttgttttatctgcattcctgcctttcatgaaagtccctcttgattgtgctgaggctgtggctcagcgaagacactgaataaatacgatagccactgttgcttgttgcttgtccaagtcttcctggcttctgctgcaagagggggatatggagaaggtgggccagggtgtgtggacccgggcagaatctggggaagaagcctgccattcgtctttctttcccacaccaccgaacccactgcccttcccacccccacagcccttttatgaaatcagacaacgtggtaggtggaaaacagcagggcctttcctctgggttttcaaccagaagtgatattccacagttttaactggttactgtgaagtccaagcggccagaattgtgaaaatgtccactgaaacactgcaagcggtgtacttaaagacagtaggccttttagattttgttatatattttttgtagtgctcttcacaagtggaaattttttttttttttttacttttttttaaaagatttttttgtaaagaagggttgtatttagaggccagtagctagagatccaaccagtggacctcttgaagcactaccaggccttaaggccaccatccgagggagactgggaaaactattattcacccaagcctccggaaatgtaatgtaccagcaggcaaaaaacagttcttcatgtagtacaaaatgaaacgaaacaaaaacaaaaacagaaagtaaaaatgaaaccaaaacatttcttaaattctagtgccatagcttttttgtttgtttgttttttgttgttgttttgttttgttcataagaaagagagaaagatactacttatccgtcagacacatgcatcctcatgtggtcgttgaactgctcgatttggtcaaactttgctgggcagacggagcagacgtaagtggtcccctccgtgcaggccaccacgcctggggggccagcgcgggcacctgggggtgtgcctgcagggggggtcccattgctggcactgtgcagggccacgtgtcgctccaggagggtcttgtgagagaacttctttttgcagatgtagcactcgtaggacttctctccccggtggaggcgcatgtgcacgttgagggagctcttctgggtgaagcgcttgttgcagatactacactggtatgccctcactcctgtgtgtgtcaccatgtgcttgataaggtaatcctttaaggagaaggagcgccaacagatgctgcattggtggggcttctcacctgtgtgtacgaacatgtgcttgacgtagttctgtttggcggtgaaagtcttgttgcagagagtgcactcataaggctttttttcgccttgcccactggctgtgctgtggcctgcggatgaggccaggggctgtggcgctggcagctgtgcagtaaaggtcgacagaccgggctgggacactgtcacaaactgggtctgctggcctgccaggggctgtggcaggctgaagaggaaaggcttggggccactgcccgcgggctgggtagtgaagagggctggcaggtaggtgttgccagctgtgccaatgacctgcgtgttgctggtcaaggtcagaggcatcctcaggttgctggtgagggtttctgtctggcgtaagtagagctgggtacttggcaatggctgcccgatggacgtgttgaccgaaggctgttgtaggacgctcttgtcggagctgttgctgacagtgataacagtgctgtccatctccacttcattgcttctctccggagaggaagcacctgtttctagctggtttgtctgcggaccaccctcagcgggggcttctgcagcctgctcgggttgggtgggttcagcctggctgtcccgcgccgccccaggcccaaactgctgctccaccgagtcaggctcggtgcctatggaggagctgacgcccgagtcgaagctttcacctttgggctcactctcggtgccctcggcctggtctgtgtcttccgtgcactcctcggattcgttgcgttccaggatctgcaccctttgctgcccgtagtagtcgtaatcgtcctccatctcctgcttgatgtggatgttgcccactagggtctggatgcgcacaggccggggctgcttgcggcagtgcgtggtctcgggggtggtggacaggtagcgctccatctgctgcgagcgctcatggatgcgtgtgatccagctggggtcttccatgtggtggtcgcggggcaggccgagcgcagtctcgtggtggctgaccactgcgccgctgtaaaaagagcgctcgccgctgccattctgcatggagcacgcgtagagtgccgagtagatcctgtccacgctgtgctgtgggtggctctgcaggtagcccgactccgtgtcgctgctctggcctgacgtgcctgactcgggagtgccccgcggcgtgtcctggcccgagtcctggatccccgggaacacatcgcccacgttctgtgacacgatgcgcgtgcactcgtcgatgactgttttgatctgcaggatgctggcggccgtgaggatctgcagagcttccgactgcgagacccgtagcacgccgctgtacatgaagtcaatgagcttttgcactgactgcactgacaccaccgacgggatctcgatgtcgctgtagccaagcagcagtttgtcctggaagaaggggctgccggctgccagcacgcagcggtgtgcgcgcagcatgctcccgtggatgcgcaccgttacgtcacagaagtggccacggttgcgctgctcgttgagggtctcgagcacggaattgctgaagttgtgaaggttgatgctgtgaatgcgctcggtcatccccttgcaactgatgtcacaatcagatgacccggtgtgagcgtgagagtttgtcagtgaatgtgttgagtggatgagggctgggtctggagacaaaacagcttcaaagttcaggcagggaaggcccggcttggcgctggatccacccggctgagtaatctcattctcctcagatgccttctggttttcagctgtcttgggtttcttcagtagtttcaaaatcaatggtgtcactcttcaggtaaattactccaaggcttgggcctagtgcagatgttcattggggcagggagcagagagcggctgcatgtaaagagaaggggcaggtcacagactgatggtcaaagatcagacagcaatgtcatgaggaatatcctgttagtaatgatgaaacattaggaatacagtgcagctcaatcttttgtttttaaggtgcagtgatttcagtctctaaatgtaacttcaggcagtctgtgcagctatggggcacaaacttgcaattcatcaattcttcagccttcagagtcccaaaggcaattcttaacacttctttttatttgtcttcttccccagcgctgagtttctcttcttataatcggtgtctccctggaagtacagtgtgagtggtaatgactgcctgcctccctaatgagtccattttcctgctcttgatgttgtgtatatacacacactgc

SEQ ID NO: 16685 - RNA, 12697 nt, Homo sapiens
  source 1..12697: mol_type = other RNA
taaaacccacaattatgtttgtctagtagaaatatatctgctggaacactttggagaacagattggtaattttgccattacactagacattagccctttcaaagcagactaagagtacgtagttccttagtgaatacaaggcttcacaactgaagagcattgcagggagcttggctaaggtgaaaagggacttgctggagaggtacagcagaatgggatgggattagaaaacaacaatctattaggaaagatgaaaggaaggaattccccagtgttcacgctgagaagtcttcatattggaccagtgtgagggggtcttttatactgaggttttaaaaacctgacttcattttgtcctgaatgtagaagtgaagaaggacactagtttcaggcacctgggatggtggaaaagtttattcaactgaggctttccatgcattgggttgaatagctgagggaagctgaagactcttatctgaaaatatgatctgaaaatatttattgtataggaagacagaatgcctgatttctgaagttttcttgatggcccaactaaagaagaaaggcaccaaatcctcactttaacaggtaaatggagatcctgagggctggatacccaagagccaccattttacggattcctcagatttaaaaatgtctcagatagatatttccaaattctatttctattagcctctgtggataaagagttcctgaaactctggttttactttttttggaaaaaaaaaaaaaaaaaaaaaaaaaaaacaactcccaggaaaatgaacactatattgccaagctgcctccagggaaaggttgaagactagttaaaataattctaagcgtattgaaaaaagaaagtgtaaagatccagtattaaaatgaatgtttgagaatacagtggggacaactaggtaattcactgtcttacgcttttcagaagactggccctttgaaacgcagcctgttattgttggtcagatcatgtggcacttaagtagccccttggtcatatttttaaaagcaaatatagacagtgacagtcctacaggggaaaatcacagatacattcatatgcacctcttttgttcttcagatattgagtgggtcagctaaacaagatcactttgaatatgaacctctttgtattagtcacaccaacaaaaaagtttcaaaaaaagttttcactttcctacatttgctaagtctgagctttaaaaaattctaaaatcctctaaagacaatactgaagctgataatataaaaagcaaattagagcactaatgattattactagatgcaccagattaactgcagcaggttggtgatgggtgatataagcaaagacataatatttcaatcaactcatgatcataggcagattcaaaagttaaaatgaatataatgtaatatatatttcaatatagagttgttatatataatgtgtatgtcctaggtttcagaaatactgcaatgtagtgtattgtagttaagtaagcatacctaaatagtaactcatattctttcacaaagtcactagtactgttaattaaaggaaaaaataaaaccgaaacaactaattgtttttccagtaaaaagaaatacctatggttacagttacagacttcttttggatatagaaagacaatatacattttaaaaagtaataacgacaaaaaagttgcaactgtaagtagccttacttaacaggggaaggggaaaagtcaccagaatagaagaggaaagaaaatgtcctctgacttctgtaaaacagaaataatgtacaaatcataaaaaataacaaaccatctagtaaaagaagggcatgggagtgagaaaactgaatcctgaattccaggccaccaaaccctcagagtccattcattcagtatattatactagagtggcattctacttcaatgcttgagatgggcaagagcaatcaattcctacagattaccaaaaaacattccccccaacagtctattggtttgctagacatggtaaacaacccactcctggaaagactttggcaaaggccacattggtttcaggagacacagtttgtgaattacgatgatatcttgtgagtacaggcagaattaggaagctttagtttgagaataaaatttatgtgtgtgtgtgtgtgtgtgtgtgtgtgtgtgcacactgcattgcatagaggaaaggaatgaagacctttgagctatgggatggctcaggccaaagtttgtgtgggctttgcctgcctggcattggtccccacccctgccacctccaggagacctggggagacgccctggactgctgctccctcttgtctgctcaccagttgaagacttctgttataccttattatggaggaaaacagcctgtccctgtgggtttgctgtggattcaacaagctgcatttgtttctcccaattctgaaacattacaaaaagcaacagagtgggcaggtgactgcttcctgggaagggagccacaagtcttaaacacaatggtgggaagaggcaactgtatctatgcacgaggacctctgcctgtgtgtgcttcctttggggggcacacacacttccagatgacaataagtatatacacaaacacacacatgtgcacacatgtcaataaatccaatagaactgtagagtttgttaaatgcactctactccacataagcatattcaagtttctcatgaaacggatacatagaaattactgatggttgggctccttcagaatgccctaaagtctcatcacagatactgatgcacccaactaaggcaacaaagcataagcagatacgtgagatatgtcagaccttcgacttctaaccagaagttcaaaaatgtatcttgttgtcactgggcaatatgaatgtgaaacagttttgtgctgagggaagctcacactgtgtgtgcacatgtataaataatgtatactcatttatagacattttggacagcagcggtgacatactggatgggttaagactctttcattattagaatctacatataaattgcaatgagtttgctgggtaaaaacaactgttgcaacactagtagaaacagatgcccccaaggtttttttttttttttttttttttttctctcttggatgtatcaaaatctcattgaggcattctaaaccaaagaaacctctgaatttgaaacagggttagtagggacttttatacccagctgggcatcccagaagcctggactctcaggactgtggctagattttgcccatgatctgtagattatgctcttgcaccggagacttgaaagttatgagtttgcattcaaacaaagaaccaccagataaaacagatgttctctaaaactgaggaaaaaaagtttagagatatacactgtatagagaaagaaagctttttgctggattgttctccttgttaaggaaatgtttaaaactagtactcccgggcacctgtgattgcattttataggattctatttagtaatatgatgtctattttacattcagccccaacctacgtcactgaaatagaataggaaatagcagccactatctgagagtacccagttctaggaaagtttggtgcctcctcaagaagtcactatttccatagtcctcaatcatgaatagggcttgtttttgtgataatgtaactattaaacagcaagaaatgcctataacttcagagccttctcatttctatatcttttatcctcttcccagggctttctgatttaaggcaataatgctacactataagtagccttttgtgaaaataccttaattgaggtcacttaagattagatttcagtctgaaagtctacagtttacggagcaaaaggtggagcctaaagaaaccactggcaggtgttttagtcagtggtgtggaaagataatgtttcttgtttcaacccagggcatttttacccatcatgcagtgaggagaaaatacatagttctgaaaaagaacccacactaggtagccctaattttctatctcttcactctaaaaaggatggaaacaagccctactgttccataaccattcccagggatcggctaaggtacattgctgactgctatagactcagtgttcaaggagaaaaaaatcttcagagacttagaaaactctttgcaatattttggtcaggctgatcgtcttgatactcagtgctagaaatgatgctttggattagtagtttccacattctgaatttataggaacactgagtcaccacagccttttttcttgtaaaggtttaagtgatatcagaaatagcaactctacacggaaagcccttgggaatatgaaaatactctctctcaagagcaagggctcttccgtgccccttttctgcctctgtatgtagcctgagcaccagggtagagattgcttttgaaagtttgccccatgtaatctatttcctggctacctaagagaacagccgttttcttcatgaaaacacaaagaggggaaagaggctgctgctgttccagtgggaagttatgtctagccccagaaggcctggtggctgggtcagctcaagcactctcttcatgcactgcaggctcaggaggcattgggttgctttgctttttctatggaattagggagcctattgaaattctagtgcacccctccttttgtttgtcaccaagtcacatggttctgtcttcagtatcctatttttctttttttttaatttctttttctgaggaacaaaattggccatttaaataaagttcttttctagtgagtaaagaggtttctcagagccagaaatcactgaaaagagagtctgtcgaccctgcccatggaaaagcccagagatttctctaaccacttcttgccaaacttcctagttttgtgattggatgtttcttggtttagcattgtttggtgctgaatacattttgcaattcttttgttctctgccctagagcttccattaccctggacttcaactcattaccaaattaaagaattcttttagaagatttcttttaagagtcaggtcacaacagaaagggcgccctcctgttctcctaaatctcaagggcatctcaggttgtgtctgctcttacgttgcaccttccttttgttcccttttaatgcagcagcacactggctatagcagaggcagacctgatttgattatctgataccttttccacaaaatcatatatcccctgctcccagccccaactaatcaaataacatcttctagaacaacagaggaaagctccagaatgggtgtatatcctgtgactcctggccagatccaccttgctccctgtcttcctaggggtcacaggtgttgggagcattgtggaggagccccaacaaggaagcaacatatggctttattatgttttctcaggaatcgaaggggttttataaggggcatatctcatttttgacttctgtgctgagagaaaatattgagttttgggcgcaggcagagcacagacaggacagctggtgttcctgtgtgagggaagtacacatagctcaaggctttaggactgaatgtgaaacaaacatacctggaggaaaacttttttcattatcagaattcacaaattcttactgttcatgggttgaaaaagagtatttgggaccttatagaatattttgatgatacaaaataaaacccttatgacttttaaacacagcaaacccaagtctttctaaggccaagagctactatgatctctaagatgactaggaatgaactgaggctagaatatgagcaggaaattatccagcacacttaatcatggcacaaatagattcaaagcattaggaatttgggaagagaacggtctataaaactgttattaggagctaaagtttacctctcaattaaaagatacaggaaaccattttgatacagagattttcatttcagattttttttctttgcttagcttgtttccccctgtgtagaattgtaacagatccatgtgttccaattattttcttttttaggattatatttcacacatttgggggccttttttgtacaaatattggcatgtaataaggaaaaattgcccatgatgctgagataataccagtgtttttagtggtagaaaatattatttttttataaaccatatctaaatatcttgagataaaaattcccctttgactttttttcctctcccttgtttggcaaattccattttaaaattataaattgctaaaaaatgtcctttccatactatttctctcttccttgtactcatcctaagaagtcttaaatctggaacatttgcttttatcttatctatctgtttcctggctactagaaagaaatttttttagcactcatatcaccctaccatgaaggtctaaatgtaagatgactgtaggacttgaaacaaaaaaaaattaaaaagatccacactcattctttgattttgaagcaaatgtctttccctatttctaaagatatttgtgattgtttaacttaaaagtgagaattgacaatctaaaagcatctctatccttttgaaacaggtccagattggtttatttcctaaaatgtgggtcagtttggaaagtggccatttgatgggccaggaacatagcaataaacaactacctctttgctcctccagattagatctcccactccaatccagcttcttcctctttccacaaaataatttgtcaactattttagaatgtgacatatttgggaaggataaatgtacagtaggaatatgtctactgctatgcaaacctggctggtccattttgtcatggactacaatgattatatcacctcattaagaattctttagggatcctccacctcctcccccactcccttttttttaagagacacttcctttacagggaaaggatgatagactcctcagggtttcaagtcacctgcagctttttctctacatgttctaccaaaagaaaaggtggattctaacccaattgcttagcattttacatggcaaatcagcattaaggcaaatgggtctctctcagatttgagaaacagaaagctacacgtggcccataatggcacctaagatcaacttttcaggcggtattagtgaaaattcttcctactttgctaaatttgaacaaagacactttcaaatctactgtgaaacagtttaaaatattttaaagtggcttttggccttctttcatttgtaacatgtattgagtgatttcatgtcattgtctcctagctttaagagtttttttcttaaggtcaatcttctcttttcattttatgggtggaatcacttgttttccaaaatatcaaaacaattccatgacatagttaattaatgctccctctattggtggtaagtggaaatattagtcttacaacactgctattttaaaaagcaaaattagcaatagaaaaatgaacttactttatctcggaagctgttcctcactaactgttaaaacagatcagttttggacatacagttcttggcaggactcctcttagaaatcacaataggttacacttaatagtcagttaaccacccaagtttacattaaaacttctagcaaaatatccactgaattaagcactgtgggaccaaatcaaactcacaaacacttcagttacactaaccttacaaagcatcacaaagaacttatgaaaaagatccaagttaaccaaatgtctaaaatatatgaataaaaccaatttagtcattacagagttgtttgtgttggaagattttccctcgtttgctgcacagtttttgtaaataaaatgctgacaggaaaattagaaggaaaattaaattaaaatgtaatgtaattttgaaactaaaatacgctctcctttcttctttttaaaactgtagtttggtgttttgctttgtttaaagatttgctttcccctaagtatgttaaaatatgcccagcaatgaaatcactttgggagtttcagctaggtttaagaattcctatatttgagctggaatcccttcaggacactgtctataatgaaaatgtctctattataacaccttgatcaggaccgaggagagaaatccctactaggaagagagagtggcatctggtatgatgcaatagattggtggtcttttgaatggtggctgttggcatctgggaatttttttgttaatttccctaaaacctttcgaagaagcaagggttaattcgtcatctaaagaatgatcatcttattcagccctcttaaccatggtggaaacagtcagaaggtgatatttggaaggaaaaaagtaattttggcatcaatgcatcttgatctataacaggcttctcataatgatgctctttgtagttgggaagggtgaggagctatggcagagttttgtgaactcctcttcctggctgatcacaaaagaaaagaccccatttatcaagacttctagactattagtgtttcactaagaaaaaaagtaaagtcaatagaaattctagaattgtaagatctcaatgaaattttggagaagcaagcaatctctttctgaaagataaagtctcttccatgaaaaagaacagaattctagatgaatcagttgaaaaaattattcagtggggcaacttaagcttgctaaagtcaaagaactacatatcaaaatacaaagcagcaattcaaattacagcagggatgggctggccacagaggccctcatcaacccaggcaatacttaaaataataaaaattaagaaaaattaaaaaaaatatgaagaaaatatccttcctctctttcaaatataactttagttgccttttattctttctatctggaagcagtatcgctaaccttaacagtcttgacttaccaaaaaatatatatatgtgtgtgaaataaaataaaagagaaggaattggtggcagtgtatgcaaaaccaaaatgaaaaaaattacttttaacaatttcactttttttgtttttttttttacacaaatactgttgtaaatatattaaaaaaatcagcattctatctggtaaacgtcacttttgcccctctataaaattttgaattaaaaaagcctcaagaactttttattgttccccccaccctccatttctttttctttttctcttccacaagaatatatcctgacactttttttttttttgcaaagattgttggaaataatccttctcttgtacctagaaacataggtgcaaatttctgatatctttgttttatctgcattcctgcctttcatgaaagtccctcttgattgtgctgaggctgtggctcagcgaagacactgaataaatacgatagccactgttgcttgttgcttgtccaagtcttcctggcttctgctgcaagagggggatatggagaaggtgggccagggtgtgtggacccgggcagaatctggggaagaagcctgccattcgtctttctttcccacaccaccgaacccactgcccttcccacccccacagcccttttatgaaatcagacaacgtggtaggtggaaaacagcagggcctttcctctgggttttcaaccagaagtgatattccacagttttaactggttactgtgaagtccaagcggccagaattgtgaaaatgtccactgaaacactgcaagcggtgtacttaaagacagtaggccttttagattttgttatatattttttgtagtgctcttcacaagtggaaattttttttttttttttacttttttttaaaagatttttttgtaaagaagggttgtatttagaggccagtagctagagatccaaccagtggacctcttgaagcactaccaggccttaaggccaccatccgagggagactgggaaaactattattcacccaagcctccggaaatgtaatgtaccagcaggcaaaaaacagttcttcatgtagtacaaaatgaaacgaaacaaaaacaaaaacagaaagtaaaaatgaaaccaaaacatttcttaaattctagtgccatagcttttttgtttgtttgttttttgttgttgttttgttttgttcataagaaagagagaaagatactacttatccgtcagacacatgcatcctcatgtggtcgttgaactgctcgatttggtcaaactttgctgggcagacggagcagacgtaagtggtcccctccgtgcaggccaccacgcctggggggccagcgcgggcacctgggggtgtgcctgcagggggggtcccattgctggcactgtgcagggccacgtgtcgctccaggagggtcttgtgagagaacttctttttgcagatgtagcactcgtaggacttctctccccggtggaggcgcatgtgcacgttgagggagctcttctgggtgaagcgcttgttgcagatactacactggtatgccctcactcctgtgtgtgtcaccatgtgcttgataaggtaatcctttaaggagaaggagcgccaacagatgctgcattggtggggcttctcacctgtgtgtacgaacatgtgcttgacgtagttctgtttggcggtgaaagtcttgttgcagagagtgcactcataaggctttttttcgccttgcccactggctgtgctgtggcctgcggatgaggccaggggctgtggcgctggcagctgtgcagtaaaggtcgacagaccgggctgggacactgtcacaaactgggtctgctggcctgccaggggctgtggcaggctgaagaggaaaggcttggggccactgcccgcgggctgggtagtgaagagggctggcaggtaggtgttgccagctgtgccaatgacctgcgtgttgctggtcaaggtcagaggcatcctcaggttgctggtgagggtttctgtctggcgtaagtagagctgggtacttggcaatggctgcccgatggacgtgttgaccgaaggctgttgtaggacgctcttgtcggagctgttgctgacagtgataacagtgctgtccatctccacttcattgcttctctccggagaggaagcacctgtttctagctggtttgtctgcggaccaccctcagcgggggcttctgcagcctgctcgggttgggtgggttcagcctggctgtcccgcgccgccccaggcccaaactgctgctccaccgagtcaggctcggtgcctatggaggagctgacgcccgagtcgaagctttcacctttgggctcactctcggtgccctcggcctggtctgtgtcttccgtgcactcctcggattcgttgcgttccaggatctgcaccctttgctgcccgtagtagtcgtaatcgtcctccatctcctgcttgatgtggatgttgcccactagggtctggatgcgcacaggccggggctgcttgcggcagtgcgtggtctcgggggtggtggacaggtagcgctccatctgctgcgagcgctcatggatgcgtgtgatccagctggggtcttccatgtggtggtcgcggggcaggccgagcgcagtctcgtggtggctgaccactgcgccgctgtaaaaagagcgctcgccgctgccattctgcatggagcacgcgtagagtgccgagtagatcctgtccacgctgtgctgtgggtggctctgcaggtagcccgactccgtgtcgctgctctggcctgacgtgcctgactcgggagtgccccgcggcgtgtcctggcccgagtcctggatccccgggaacacatcgcccacgttctgtgacacgatgcgcgtgcactcgtcgatgactgttttgatctgcaggatgctggcggccgtgaggatctgcagagcttccgactgcgagacccgtagcacgccgctgtacatgaagtcaatgagcttttgcactgactgcactgacaccaccgacgggatctcgatgtcgctgtagccaagcagcagtttgtcctggaagaaggggctgccggctgccagcacgcagcggtgtgcgcgcagcatgctcccgtggatgcgcaccgttacgtcacagaagtggccacggttgcgctgctcgttgagggtctcgagcacggaattgctgaagttgtgaaggttgatgctgtgaatgcgctcggtcatccccttgcaactgatgtcacaatcagatgacccggtgtgagcgtgagagtttgtcagtgaatgtgttgagtggatgagggctgggtctggagacaaaacagcttcaaagttcaggcagggaaggcccggcttggcgctggatccacccggctgagtaatctcattctcctcagatgccttctggttttcagctgtcttgggtttcttcagtagtttcaaaatcaatggtgtcactcttcaggtaaattactccaaggcttgggcctagtgcagatgttcattggggcagggagcagagagcggctgcatgtaaagagaaggggcaggtcacagactgatggtcaaagatcagacagcaatgtcatgaggaatatcctgttagtaatgatgaaacattctccaaacattctcagagttcattcttcgtaccctgtaggcttatgctgcacaagtctgaaacatcagtctatgtattttttttgaaatgtactctgtaccgatgcatttttctgtgtttctttctaaccctcgagaatgttaagaatttaggaagagagccacagcttaagagtgcaattatttgccagtaaatactcaatttgcttgtcctgtgatttttcttctaacttgcatattcaataatccgtccctgact

SEQ ID NO: 16686 - RNA, 12759 nt, Homo sapiens
  source 1..12759: mol_type = other RNA
taaaacccacaattatgtttgtctagtagaaatatatctgctggaacactttggagaacagattggtaattttgccattacactagacattagccctttcaaagcagactaagagtacgtagttccttagtgaatacaaggcttcacaactgaagagcattgcagggagcttggctaaggtgaaaagggacttgctggagaggtacagcagaatgggatgggattagaaaacaacaatctattaggaaagatgaaaggaaggaattccccagtgttcacgctgagaagtcttcatattggaccagtgtgagggggtcttttatactgaggttttaaaaacctgacttcattttgtcctgaatgtagaagtgaagaaggacactagtttcaggcacctgggatggtggaaaagtttattcaactgaggctttccatgcattgggttgaatagctgagggaagctgaagactcttatctgaaaatatgatctgaaaatatttattgtataggaagacagaatgcctgatttctgaagttttcttgatggcccaactaaagaagaaaggcaccaaatcctcactttaacaggtaaatggagatcctgagggctggatacccaagagccaccattttacggattcctcagatttaaaaatgtctcagatagatatttccaaattctatttctattagcctctgtggataaagagttcctgaaactctggttttactttttttggaaaaaaaaaaaaaaaaaaaaaaaaaaaacaactcccaggaaaatgaacactatattgccaagctgcctccagggaaaggttgaagactagttaaaataattctaagcgtattgaaaaaagaaagtgtaaagatccagtattaaaatgaatgtttgagaatacagtggggacaactaggtaattcactgtcttacgcttttcagaagactggccctttgaaacgcagcctgttattgttggtcagatcatgtggcacttaagtagccccttggtcatatttttaaaagcaaatatagacagtgacagtcctacaggggaaaatcacagatacattcatatgcacctcttttgttcttcagatattgagtgggtcagctaaacaagatcactttgaatatgaacctctttgtattagtcacaccaacaaaaaagtttcaaaaaaagttttcactttcctacatttgctaagtctgagctttaaaaaattctaaaatcctctaaagacaatactgaagctgataatataaaaagcaaattagagcactaatgattattactagatgcaccagattaactgcagcaggttggtgatgggtgatataagcaaagacataatatttcaatcaactcatgatcataggcagattcaaaagttaaaatgaatataatgtaatatatatttcaatatagagttgttatatataatgtgtatgtcctaggtttcagaaatactgcaatgtagtgtattgtagttaagtaagcatacctaaatagtaactcatattctttcacaaagtcactagtactgttaattaaaggaaaaaataaaaccgaaacaactaattgtttttccagtaaaaagaaatacctatggttacagttacagacttcttttggatatagaaagacaatatacattttaaaaagtaataacgacaaaaaagttgcaactgtaagtagccttacttaacaggggaaggggaaaagtcaccagaatagaagaggaaagaaaatgtcctctgacttctgtaaaacagaaataatgtacaaatcataaaaaataacaaaccatctagtaaaagaagggcatgggagtgagaaaactgaatcctgaattccaggccaccaaaccctcagagtccattcattcagtatattatactagagtggcattctacttcaatgcttgagatgggcaagagcaatcaattcctacagattaccaaaaaacattccccccaacagtctattggtttgctagacatggtaaacaacccactcctggaaagactttggcaaaggccacattggtttcaggagacacagtttgtgaattacgatgatatcttgtgagtacaggcagaattaggaagctttagtttgagaataaaatttatgtgtgtgtgtgtgtgtgtgtgtgtgtgtgtgcacactgcattgcatagaggaaaggaatgaagacctttgagctatgggatggctcaggccaaagtttgtgtgggctttgcctgcctggcattggtccccacccctgccacctccaggagacctggggagacgccctggactgctgctccctcttgtctgctcaccagttgaagacttctgttataccttattatggaggaaaacagcctgtccctgtgggtttgctgtggattcaacaagctgcatttgtttctcccaattctgaaacattacaaaaagcaacagagtgggcaggtgactgcttcctgggaagggagccacaagtcttaaacacaatggtgggaagaggcaactgtatctatgcacgaggacctctgcctgtgtgtgcttcctttggggggcacacacacttccagatgacaataagtatatacacaaacacacacatgtgcacacatgtcaataaatccaatagaactgtagagtttgttaaatgcactctactccacataagcatattcaagtttctcatgaaacggatacatagaaattactgatggttgggctccttcagaatgccctaaagtctcatcacagatactgatgcacccaactaaggcaacaaagcataagcagatacgtgagatatgtcagaccttcgacttctaaccagaagttcaaaaatgtatcttgttgtcactgggcaatatgaatgtgaaacagttttgtgctgagggaagctcacactgtgtgtgcacatgtataaataatgtatactcatttatagacattttggacagcagcggtgacatactggatgggttaagactctttcattattagaatctacatataaattgcaatgagtttgctgggtaaaaacaactgttgcaacactagtagaaacagatgcccccaaggtttttttttttttttttttttttttctctcttggatgtatcaaaatctcattgaggcattctaaaccaaagaaacctctgaatttgaaacagggttagtagggacttttatacccagctgggcatcccagaagcctggactctcaggactgtggctagattttgcccatgatctgtagattatgctcttgcaccggagacttgaaagttatgagtttgcattcaaacaaagaaccaccagataaaacagatgttctctaaaactgaggaaaaaaagtttagagatatacactgtatagagaaagaaagctttttgctggattgttctccttgttaaggaaatgtttaaaactagtactcccgggcacctgtgattgcattttataggattctatttagtaatatgatgtctattttacattcagccccaacctacgtcactgaaatagaataggaaatagcagccactatctgagagtacccagttctaggaaagtttggtgcctcctcaagaagtcactatttccatagtcctcaatcatgaatagggcttgtttttgtgataatgtaactattaaacagcaagaaatgcctataacttcagagccttctcatttctatatcttttatcctcttcccagggctttctgatttaaggcaataatgctacactataagtagccttttgtgaaaataccttaattgaggtcacttaagattagatttcagtctgaaagtctacagtttacggagcaaaaggtggagcctaaagaaaccactggcaggtgttttagtcagtggtgtggaaagataatgtttcttgtttcaacccagggcatttttacccatcatgcagtgaggagaaaatacatagttctgaaaaagaacccacactaggtagccctaattttctatctcttcactctaaaaaggatggaaacaagccctactgttccataaccattcccagggatcggctaaggtacattgctgactgctatagactcagtgttcaaggagaaaaaaatcttcagagacttagaaaactctttgcaatattttggtcaggctgatcgtcttgatactcagtgctagaaatgatgctttggattagtagtttccacattctgaatttataggaacactgagtcaccacagccttttttcttgtaaaggtttaagtgatatcagaaatagcaactctacacggaaagcccttgggaatatgaaaatactctctctcaagagcaagggctcttccgtgccccttttctgcctctgtatgtagcctgagcaccagggtagagattgcttttgaaagtttgccccatgtaatctatttcctggctacctaagagaacagccgttttcttcatgaaaacacaaagaggggaaagaggctgctgctgttccagtgggaagttatgtctagccccagaaggcctggtggctgggtcagctcaagcactctcttcatgcactgcaggctcaggaggcattgggttgctttgctttttctatggaattagggagcctattgaaattctagtgcacccctccttttgtttgtcaccaagtcacatggttctgtcttcagtatcctatttttctttttttttaatttctttttctgaggaacaaaattggccatttaaataaagttcttttctagtgagtaaagaggtttctcagagccagaaatcactgaaaagagagtctgtcgaccctgcccatggaaaagcccagagatttctctaaccacttcttgccaaacttcctagttttgtgattggatgtttcttggtttagcattgtttggtgctgaatacattttgcaattcttttgttctctgccctagagcttccattaccctggacttcaactcattaccaaattaaagaattcttttagaagatttcttttaagagtcaggtcacaacagaaagggcgccctcctgttctcctaaatctcaagggcatctcaggttgtgtctgctcttacgttgcaccttccttttgttcccttttaatgcagcagcacactggctatagcagaggcagacctgatttgattatctgataccttttccacaaaatcatatatcccctgctcccagccccaactaatcaaataacatcttctagaacaacagaggaaagctccagaatgggtgtatatcctgtgactcctggccagatccaccttgctccctgtcttcctaggggtcacaggtgttgggagcattgtggaggagccccaacaaggaagcaacatatggctttattatgttttctcaggaatcgaaggggttttataaggggcatatctcatttttgacttctgtgctgagagaaaatattgagttttgggcgcaggcagagcacagacaggacagctggtgttcctgtgtgagggaagtacacatagctcaaggctttaggactgaatgtgaaacaaacatacctggaggaaaacttttttcattatcagaattcacaaattcttactgttcatgggttgaaaaagagtatttgggaccttatagaatattttgatgatacaaaataaaacccttatgacttttaaacacagcaaacccaagtctttctaaggccaagagctactatgatctctaagatgactaggaatgaactgaggctagaatatgagcaggaaattatccagcacacttaatcatggcacaaatagattcaaagcattaggaatttgggaagagaacggtctataaaactgttattaggagctaaagtttacctctcaattaaaagatacaggaaaccattttgatacagagattttcatttcagattttttttctttgcttagcttgtttccccctgtgtagaattgtaacagatccatgtgttccaattattttcttttttaggattatatttcacacatttgggggccttttttgtacaaatattggcatgtaataaggaaaaattgcccatgatgctgagataataccagtgtttttagtggtagaaaatattatttttttataaaccatatctaaatatcttgagataaaaattcccctttgactttttttcctctcccttgtttggcaaattccattttaaaattataaattgctaaaaaatgtcctttccatactatttctctcttccttgtactcatcctaagaagtcttaaatctggaacatttgcttttatcttatctatctgtttcctggctactagaaagaaatttttttagcactcatatcaccctaccatgaaggtctaaatgtaagatgactgtaggacttgaaacaaaaaaaaattaaaaagatccacactcattctttgattttgaagcaaatgtctttccctatttctaaagatatttgtgattgtttaacttaaaagtgagaattgacaatctaaaagcatctctatccttttgaaacaggtccagattggtttatttcctaaaatgtgggtcagtttggaaagtggccatttgatgggccaggaacatagcaataaacaactacctctttgctcctccagattagatctcccactccaatccagcttcttcctctttccacaaaataatttgtcaactattttagaatgtgacatatttgggaaggataaatgtacagtaggaatatgtctactgctatgcaaacctggctggtccattttgtcatggactacaatgattatatcacctcattaagaattctttagggatcctccacctcctcccccactcccttttttttaagagacacttcctttacagggaaaggatgatagactcctcagggtttcaagtcacctgcagctttttctctacatgttctaccaaaagaaaaggtggattctaacccaattgcttagcattttacatggcaaatcagcattaaggcaaatgggtctctctcagatttgagaaacagaaagctacacgtggcccataatggcacctaagatcaacttttcaggcggtattagtgaaaattcttcctactttgctaaatttgaacaaagacactttcaaatctactgtgaaacagtttaaaatattttaaagtggcttttggccttctttcatttgtaacatgtattgagtgatttcatgtcattgtctcctagctttaagagtttttttcttaaggtcaatcttctcttttcattttatgggtggaatcacttgttttccaaaatatcaaaacaattccatgacatagttaattaatgctccctctattggtggtaagtggaaatattagtcttacaacactgctattttaaaaagcaaaattagcaatagaaaaatgaacttactttatctcggaagctgttcctcactaactgttaaaacagatcagttttggacatacagttcttggcaggactcctcttagaaatcacaataggttacacttaatagtcagttaaccacccaagtttacattaaaacttctagcaaaatatccactgaattaagcactgtgggaccaaatcaaactcacaaacacttcagttacactaaccttacaaagcatcacaaagaacttatgaaaaagatccaagttaaccaaatgtctaaaatatatgaataaaaccaatttagtcattacagagttgtttgtgttggaagattttccctcgtttgctgcacagtttttgtaaataaaatgctgacaggaaaattagaaggaaaattaaattaaaatgtaatgtaattttgaaactaaaatacgctctcctttcttctttttaaaactgtagtttggtgttttgctttgtttaaagatttgctttcccctaagtatgttaaaatatgcccagcaatgaaatcactttgggagtttcagctaggtttaagaattcctatatttgagctggaatcccttcaggacactgtctataatgaaaatgtctctattataacaccttgatcaggaccgaggagagaaatccctactaggaagagagagtggcatctggtatgatgcaatagattggtggtcttttgaatggtggctgttggcatctgggaatttttttgttaatttccctaaaacctttcgaagaagcaagggttaattcgtcatctaaagaatgatcatcttattcagccctcttaaccatggtggaaacagtcagaaggtgatatttggaaggaaaaaagtaattttggcatcaatgcatcttgatctataacaggcttctcataatgatgctctttgtagttgggaagggtgaggagctatggcagagttttgtgaactcctcttcctggctgatcacaaaagaaaagaccccatttatcaagacttctagactattagtgtttcactaagaaaaaaagtaaagtcaatagaaattctagaattgtaagatctcaatgaaattttggagaagcaagcaatctctttctgaaagataaagtctcttccatgaaaaagaacagaattctagatgaatcagttgaaaaaattattcagtggggcaacttaagcttgctaaagtcaaagaactacatatcaaaatacaaagcagcaattcaaattacagcagggatgggctggccacagaggccctcatcaacccaggcaatacttaaaataataaaaattaagaaaaattaaaaaaaatatgaagaaaatatccttcctctctttcaaatataactttagttgccttttattctttctatctggaagcagtatcgctaaccttaacagtcttgacttaccaaaaaatatatatatgtgtgtgaaataaaataaaagagaaggaattggtggcagtgtatgcaaaaccaaaatgaaaaaaattacttttaacaatttcactttttttgtttttttttttacacaaatactgttgtaaatatattaaaaaaatcagcattctatctggtaaacgtcacttttgcccctctataaaattttgaattaaaaaagcctcaagaactttttattgttccccccaccctccatttctttttctttttctcttccacaagaatatatcctgacactttttttttttttgcaaagattgttggaaataatccttctcttgtacctagaaacataggtgcaaatttctgatatctttgttttatctgcattcctgcctttcatgaaagtccctcttgattgtgctgaggctgtggctcagcgaagacactgaataaatacgatagccactgttgcttgttgcttgtccaagtcttcctggcttctgctgcaagagggggatatggagaaggtgggccagggtgtgtggacccgggcagaatctggggaagaagcctgccattcgtctttctttcccacaccaccgaacccactgcccttcccacccccacagcccttttatgaaatcagacaacgtggtaggtggaaaacagcagggcctttcctctgggttttcaaccagaagtgatattccacagttttaactggttactgtgaagtccaagcggccagaattgtgaaaatgtccactgaaacactgcaagcggtgtacttaaagacagtaggccttttagattttgttatatattttttgtagtgctcttcacaagtggaaattttttttttttttttacttttttttaaaagatttttttgtaaagaagggttgtatttagaggccagtagctagagatccaaccagtggacctcttgaagcactaccaggccttaaggccaccatccgagggagactgggaaaactattattcacccaagcctccggaaatgtaatgtaccagcaggcaaaaaacagttcttcatgtagtacaaaatgaaacgaaacaaaaacaaaaacagaaagtaaaaatgaaaccaaaacatttcttaaattctagtgccatagcttttttgtttgtttgttttttgttgttgttttgttttgttcataagaaagagagaaagatactacttatccgtcagacacatgcatcctcatgtggtcgttgaactgctcgatttggtcaaactttgctgggcagacggagcagacgtaagtggtcccctccgtgcaggccaccacgcctggggggccagcgcgggcacctgggggtgtgcctgcagggggggtcccattgctggcactgtgcagggccacgtgtcgctccaggagggtcttgtgagagaacttctttttgcagatgtagcactcgtaggacttctctccccggtggaggcgcatgtgcacgttgagggagctcttctgggtgaagcgcttgttgcagatactacactggtatgccctcactcctgtgtgtgtcaccatgtgcttgataaggtaatcctttaaggagaaggagcgccaacagatgctgcattggtggggcttctcacctgtgtgtacgaacatgtgcttgacgtagttctgtttggcggtgaaagtcttgttgcagagagtgcactcataaggctttttttcgccttgcccactggctgtgctgtggcctgcggatgaggccaggggctgtggcgctggcagctgtgcagtaaaggtcgacagaccgggctgggacactgtcacaaactgggtctgctggcctgccaggggctgtggcaggctgaagaggaaaggcttggggccactgcccgcgggctgggtagtgaagagggctggcaggtaggtgttgccagctgtgccaatgacctgcgtgttgctggtcaaggtcagaggcatcctcaggttgctggtgagggtttctgtctggcgtaagtagagctgggtacttggcaatggctgcccgatggacgtgttgaccgaaggctgttgtaggacgctcttgtcggagctgttgctgacagtgataacagtgctgtccatctccacttcattgcttctctccggagaggaagcacctgtttctagctggtttgtctgcggaccaccctcagcgggggcttctgcagcctgctcgggttgggtgggttcagcctggctgtcccgcgccgccccaggcccaaactgctgctccaccgagtcaggctcggtgcctatggaggagctgacgcccgagtcgaagctttcacctttgggctcactctcggtgccctcggcctggtctgtgtcttccgtgcactcctcggattcgttgcgttccaggatctgcaccctttgctgcccgtagtagtcgtaatcgtcctccatctcctgcttgatgtggatgttgcccactagggtctggatgcgcacaggccggggctgcttgcggcagtgcgtggtctcgggggtggtggacaggtagcgctccatctgctgcgagcgctcatggatgcgtgtgatccagctggggtcttccatgtggtggtcgcggggcaggccgagcgcagtctcgtggtggctgaccactgcgccgctgtaaaaagagcgctcgccgctgccattctgcatggagcacgcgtagagtgccgagtagatcctgtccacgctgtgctgtgggtggctctgcaggtagcccgactccgtgtcgctgctctggcctgacgtgcctgactcgggagtgccccgcggcgtgtcctggcccgagtcctggatccccgggaacacatcgcccacgttctgtgacacgatgcgcgtgcactcgtcgatgactgttttgatctgcaggatgctggcggccgtgaggatctgcagagcttccgactgcgagacccgtagcacgccgctgtacatgaagtcaatgagcttttgcactgactgcactgacaccaccgacgggatctcgatgtcgctgtagccaagcagcagtttgtcctggaagaaggggctgccggctgccagcacgcagcggtgtgcgcgcagcatgctcccgtggatgcgcaccgttacgtcacagaagtggccacggttgcgctgctcgttgagggtctcgagcacggaattgctgaagttgtgaaggttgatgctgtgaatgcgctcggtcatccccttgcaactgatgtcacaatcagatgacccggtgtgagcgtgagagtttgtcagtgaatgtgttgagtggatgagggctgggtctggagacaaaacagcttcaaagttcaggcagggaaggcccggcttggcgctggatccacccggctgagtaatctcattctcctcagatgccttctggttttcagctgtcttgggtttcttcagtagtttcaaaatcaatggtgtcactcttcaggtaaattactccaaggcttgggcctagtgcagatgttcattggggcagggagcagagagcggctgcatgtaaagagaaggggcaggtcacagactgatggtcaaagatcagacagcaatgtcatgaggaatatcctgttagtaatgatgaaacattctccaaacattctcagagttcattcttcgtaccctgtaggcttatgctgtgaaataggtaataggaagccttggtaggtgctttccaggaatacagtgcagctcaatcttttgtttttaaggtgcagtgatttcagtctctaaatgtaacttcaggcagtctgtgcagctatggggcacaaacttgcaattcatcaattcttcagccttcagagtcccaaaggcaattcttaacacttctttttatttgtctcctcgcgctctttaatcttctttcctcaactcctaaacttccccccgcccctacttcttcggcagaag

SEQ ID NO: 16687 - RNA, 12651 nt, Homo sapiens
  source 1..12651: mol_type = other RNA
taaaacccacaattatgtttgtctagtagaaatatatctgctggaacactttggagaacagattggtaattttgccattacactagacattagccctttcaaagcagactaagagtacgtagttccttagtgaatacaaggcttcacaactgaagagcattgcagggagcttggctaaggtgaaaagggacttgctggagaggtacagcagaatgggatgggattagaaaacaacaatctattaggaaagatgaaaggaaggaattccccagtgttcacgctgagaagtcttcatattggaccagtgtgagggggtcttttatactgaggttttaaaaacctgacttcattttgtcctgaatgtagaagtgaagaaggacactagtttcaggcacctgggatggtggaaaagtttattcaactgaggctttccatgcattgggttgaatagctgagggaagctgaagactcttatctgaaaatatgatctgaaaatatttattgtataggaagacagaatgcctgatttctgaagttttcttgatggcccaactaaagaagaaaggcaccaaatcctcactttaacaggtaaatggagatcctgagggctggatacccaagagccaccattttacggattcctcagatttaaaaatgtctcagatagatatttccaaattctatttctattagcctctgtggataaagagttcctgaaactctggttttactttttttggaaaaaaaaaaaaaaaaaaaaaaaaaaaacaactcccaggaaaatgaacactatattgccaagctgcctccagggaaaggttgaagactagttaaaataattctaagcgtattgaaaaaagaaagtgtaaagatccagtattaaaatgaatgtttgagaatacagtggggacaactaggtaattcactgtcttacgcttttcagaagactggccctttgaaacgcagcctgttattgttggtcagatcatgtggcacttaagtagccccttggtcatatttttaaaagcaaatatagacagtgacagtcctacaggggaaaatcacagatacattcatatgcacctcttttgttcttcagatattgagtgggtcagctaaacaagatcactttgaatatgaacctctttgtattagtcacaccaacaaaaaagtttcaaaaaaagttttcactttcctacatttgctaagtctgagctttaaaaaattctaaaatcctctaaagacaatactgaagctgataatataaaaagcaaattagagcactaatgattattactagatgcaccagattaactgcagcaggttggtgatgggtgatataagcaaagacataatatttcaatcaactcatgatcataggcagattcaaaagttaaaatgaatataatgtaatatatatttcaatatagagttgttatatataatgtgtatgtcctaggtttcagaaatactgcaatgtagtgtattgtagttaagtaagcatacctaaatagtaactcatattctttcacaaagtcactagtactgttaattaaaggaaaaaataaaaccgaaacaactaattgtttttccagtaaaaagaaatacctatggttacagttacagacttcttttggatatagaaagacaatatacattttaaaaagtaataacgacaaaaaagttgcaactgtaagtagccttacttaacaggggaaggggaaaagtcaccagaatagaagaggaaagaaaatgtcctctgacttctgtaaaacagaaataatgtacaaatcataaaaaataacaaaccatctagtaaaagaagggcatgggagtgagaaaactgaatcctgaattccaggccaccaaaccctcagagtccattcattcagtatattatactagagtggcattctacttcaatgcttgagatgggcaagagcaatcaattcctacagattaccaaaaaacattccccccaacagtctattggtttgctagacatggtaaacaacccactcctggaaagactttggcaaaggccacattggtttcaggagacacagtttgtgaattacgatgatatcttgtgagtacaggcagaattaggaagctttagtttgagaataaaatttatgtgtgtgtgtgtgtgtgtgtgtgtgtgtgtgcacactgcattgcatagaggaaaggaatgaagacctttgagctatgggatggctcaggccaaagtttgtgtgggctttgcctgcctggcattggtccccacccctgccacctccaggagacctggggagacgccctggactgctgctccctcttgtctgctcaccagttgaagacttctgttataccttattatggaggaaaacagcctgtccctgtgggtttgctgtggattcaacaagctgcatttgtttctcccaattctgaaacattacaaaaagcaacagagtgggcaggtgactgcttcctgggaagggagccacaagtcttaaacacaatggtgggaagaggcaactgtatctatgcacgaggacctctgcctgtgtgtgcttcctttggggggcacacacacttccagatgacaataagtatatacacaaacacacacatgtgcacacatgtcaataaatccaatagaactgtagagtttgttaaatgcactctactccacataagcatattcaagtttctcatgaaacggatacatagaaattactgatggttgggctccttcagaatgccctaaagtctcatcacagatactgatgcacccaactaaggcaacaaagcataagcagatacgtgagatatgtcagaccttcgacttctaaccagaagttcaaaaatgtatcttgttgtcactgggcaatatgaatgtgaaacagttttgtgctgagggaagctcacactgtgtgtgcacatgtataaataatgtatactcatttatagacattttggacagcagcggtgacatactggatgggttaagactctttcattattagaatctacatataaattgcaatgagtttgctgggtaaaaacaactgttgcaacactagtagaaacagatgcccccaaggtttttttttttttttttttttttttctctcttggatgtatcaaaatctcattgaggcattctaaaccaaagaaacctctgaatttgaaacagggttagtagggacttttatacccagctgggcatcccagaagcctggactctcaggactgtggctagattttgcccatgatctgtagattatgctcttgcaccggagacttgaaagttatgagtttgcattcaaacaaagaaccaccagataaaacagatgttctctaaaactgaggaaaaaaagtttagagatatacactgtatagagaaagaaagctttttgctggattgttctccttgttaaggaaatgtttaaaactagtactcccgggcacctgtgattgcattttataggattctatttagtaatatgatgtctattttacattcagccccaacctacgtcactgaaatagaataggaaatagcagccactatctgagagtacccagttctaggaaagtttggtgcctcctcaagaagtcactatttccatagtcctcaatcatgaatagggcttgtttttgtgataatgtaactattaaacagcaagaaatgcctataacttcagagccttctcatttctatatcttttatcctcttcccagggctttctgatttaaggcaataatgctacactataagtagccttttgtgaaaataccttaattgaggtcacttaagattagatttcagtctgaaagtctacagtttacggagcaaaaggtggagcctaaagaaaccactggcaggtgttttagtcagtggtgtggaaagataatgtttcttgtttcaacccagggcatttttacccatcatgcagtgaggagaaaatacatagttctgaaaaagaacccacactaggtagccctaattttctatctcttcactctaaaaaggatggaaacaagccctactgttccataaccattcccagggatcggctaaggtacattgctgactgctatagactcagtgttcaaggagaaaaaaatcttcagagacttagaaaactctttgcaatattttggtcaggctgatcgtcttgatactcagtgctagaaatgatgctttggattagtagtttccacattctgaatttataggaacactgagtcaccacagccttttttcttgtaaaggtttaagtgatatcagaaatagcaactctacacggaaagcccttgggaatatgaaaatactctctctcaagagcaagggctcttccgtgccccttttctgcctctgtatgtagcctgagcaccagggtagagattgcttttgaaagtttgccccatgtaatctatttcctggctacctaagagaacagccgttttcttcatgaaaacacaaagaggggaaagaggctgctgctgttccagtgggaagttatgtctagccccagaaggcctggtggctgggtcagctcaagcactctcttcatgcactgcaggctcaggaggcattgggttgctttgctttttctatggaattagggagcctattgaaattctagtgcacccctccttttgtttgtcaccaagtcacatggttctgtcttcagtatcctatttttctttttttttaatttctttttctgaggaacaaaattggccatttaaataaagttcttttctagtgagtaaagaggtttctcagagccagaaatcactgaaaagagagtctgtcgaccctgcccatggaaaagcccagagatttctctaaccacttcttgccaaacttcctagttttgtgattggatgtttcttggtttagcattgtttggtgctgaatacattttgcaattcttttgttctctgccctagagcttccattaccctggacttcaactcattaccaaattaaagaattcttttagaagatttcttttaagagtcaggtcacaacagaaagggcgccctcctgttctcctaaatctcaagggcatctcaggttgtgtctgctcttacgttgcaccttccttttgttcccttttaatgcagcagcacactggctatagcagaggcagacctgatttgattatctgataccttttccacaaaatcatatatcccctgctcccagccccaactaatcaaataacatcttctagaacaacagaggaaagctccagaatgggtgtatatcctgtgactcctggccagatccaccttgctccctgtcttcctaggggtcacaggtgttgggagcattgtggaggagccccaacaaggaagcaacatatggctttattatgttttctcaggaatcgaaggggttttataaggggcatatctcatttttgacttctgtgctgagagaaaatattgagttttgggcgcaggcagagcacagacaggacagctggtgttcctgtgtgagggaagtacacatagctcaaggctttaggactgaatgtgaaacaaacatacctggaggaaaacttttttcattatcagaattcacaaattcttactgttcatgggttgaaaaagagtatttgggaccttatagaatattttgatgatacaaaataaaacccttatgacttttaaacacagcaaacccaagtctttctaaggccaagagctactatgatctctaagatgactaggaatgaactgaggctagaatatgagcaggaaattatccagcacacttaatcatggcacaaatagattcaaagcattaggaatttgggaagagaacggtctataaaactgttattaggagctaaagtttacctctcaattaaaagatacaggaaaccattttgatacagagattttcatttcagattttttttctttgcttagcttgtttccccctgtgtagaattgtaacagatccatgtgttccaattattttcttttttaggattatatttcacacatttgggggccttttttgtacaaatattggcatgtaataaggaaaaattgcccatgatgctgagataataccagtgtttttagtggtagaaaatattatttttttataaaccatatctaaatatcttgagataaaaattcccctttgactttttttcctctcccttgtttggcaaattccattttaaaattataaattgctaaaaaatgtcctttccatactatttctctcttccttgtactcatcctaagaagtcttaaatctggaacatttgcttttatcttatctatctgtttcctggctactagaaagaaatttttttagcactcatatcaccctaccatgaaggtctaaatgtaagatgactgtaggacttgaaacaaaaaaaaattaaaaagatccacactcattctttgattttgaagcaaatgtctttccctatttctaaagatatttgtgattgtttaacttaaaagtgagaattgacaatctaaaagcatctctatccttttgaaacaggtccagattggtttatttcctaaaatgtgggtcagtttggaaagtggccatttgatgggccaggaacatagcaataaacaactacctctttgctcctccagattagatctcccactccaatccagcttcttcctctttccacaaaataatttgtcaactattttagaatgtgacatatttgggaaggataaatgtacagtaggaatatgtctactgctatgcaaacctggctggtccattttgtcatggactacaatgattatatcacctcattaagaattctttagggatcctccacctcctcccccactcccttttttttaagagacacttcctttacagggaaaggatgatagactcctcagggtttcaagtcacctgcagctttttctctacatgttctaccaaaagaaaaggtggattctaacccaattgcttagcattttacatggcaaatcagcattaaggcaaatgggtctctctcagatttgagaaacagaaagctacacgtggcccataatggcacctaagatcaacttttcaggcggtattagtgaaaattcttcctactttgctaaatttgaacaaagacactttcaaatctactgtgaaacagtttaaaatattttaaagtggcttttggccttctttcatttgtaacatgtattgagtgatttcatgtcattgtctcctagctttaagagtttttttcttaaggtcaatcttctcttttcattttatgggtggaatcacttgttttccaaaatatcaaaacaattccatgacatagttaattaatgctccctctattggtggtaagtggaaatattagtcttacaacactgctattttaaaaagcaaaattagcaatagaaaaatgaacttactttatctcggaagctgttcctcactaactgttaaaacagatcagttttggacatacagttcttggcaggactcctcttagaaatcacaataggttacacttaatagtcagttaaccacccaagtttacattaaaacttctagcaaaatatccactgaattaagcactgtgggaccaaatcaaactcacaaacacttcagttacactaaccttacaaagcatcacaaagaacttatgaaaaagatccaagttaaccaaatgtctaaaatatatgaataaaaccaatttagtcattacagagttgtttgtgttggaagattttccctcgtttgctgcacagtttttgtaaataaaatgctgacaggaaaattagaaggaaaattaaattaaaatgtaatgtaattttgaaactaaaatacgctctcctttcttctttttaaaactgtagtttggtgttttgctttgtttaaagatttgctttcccctaagtatgttaaaatatgcccagcaatgaaatcactttgggagtttcagctaggtttaagaattcctatatttgagctggaatcccttcaggacactgtctataatgaaaatgtctctattataacaccttgatcaggaccgaggagagaaatccctactaggaagagagagtggcatctggtatgatgcaatagattggtggtcttttgaatggtggctgttggcatctgggaatttttttgttaatttccctaaaacctttcgaagaagcaagggttaattcgtcatctaaagaatgatcatcttattcagccctcttaaccatggtggaaacagtcagaaggtgatatttggaaggaaaaaagtaattttggcatcaatgcatcttgatctataacaggcttctcataatgatgctctttgtagttgggaagggtgaggagctatggcagagttttgtgaactcctcttcctggctgatcacaaaagaaaagaccccatttatcaagacttctagactattagtgtttcactaagaaaaaaagtaaagtcaatagaaattctagaattgtaagatctcaatgaaattttggagaagcaagcaatctctttctgaaagataaagtctcttccatgaaaaagaacagaattctagatgaatcagttgaaaaaattattcagtggggcaacttaagcttgctaaagtcaaagaactacatatcaaaatacaaagcagcaattcaaattacagcagggatgggctggccacagaggccctcatcaacccaggcaatacttaaaataataaaaattaagaaaaattaaaaaaaatatgaagaaaatatccttcctctctttcaaatataactttagttgccttttattctttctatctggaagcagtatcgctaaccttaacagtcttgacttaccaaaaaatatatatatgtgtgtgaaataaaataaaagagaaggaattggtggcagtgtatgcaaaaccaaaatgaaaaaaattacttttaacaatttcactttttttgtttttttttttacacaaatactgttgtaaatatattaaaaaaatcagcattctatctggtaaacgtcacttttgcccctctataaaattttgaattaaaaaagcctcaagaactttttattgttccccccaccctccatttctttttctttttctcttccacaagaatatatcctgacactttttttttttttgcaaagattgttggaaataatccttctcttgtacctagaaacataggtgcaaatttctgatatctttgttttatctgcattcctgcctttcatgaaagtccctcttgattgtgctgaggctgtggctcagcgaagacactgaataaatacgatagccactgttgcttgttgcttgtccaagtcttcctggcttctgctgcaagagggggatatggagaaggtgggccagggtgtgtggacccgggcagaatctggggaagaagcctgccattcgtctttctttcccacaccaccgaacccactgcccttcccacccccacagcccttttatgaaatcagacaacgtggtaggtggaaaacagcagggcctttcctctgggttttcaaccagaagtgatattccacagttttaactggttactgtgaagtccaagcggccagaattgtgaaaatgtccactgaaacactgcaagcggtgtacttaaagacagtaggccttttagattttgttatatattttttgtagtgctcttcacaagtggaaattttttttttttttttacttttttttaaaagatttttttgtaaagaagggttgtatttagaggccagtagctagagatccaaccagtggacctcttgaagcactaccaggccttaaggccaccatccgagggagactgggaaaactattattcacccaagcctccggaaatgtaatgtaccagcaggcaaaaaacagttcttcatgtagtacaaaatgaaacgaaacaaaaacaaaaacagaaagtaaaaatgaaaccaaaacatttcttaaattctagtgccatagcttttttgtttgtttgttttttgttgttgttttgttttgttcataagaaagagagaaagatactacttatccgtcagacacatgcatcctcatgtggtcgttgaactgctcgatttggtcaaactttgctgggcagacggagcagacgtaagtggtcccctccgtgcaggccaccacgcctggggggccagcgcgggcacctgggggtgtgcctgcagggggggtcccattgctggcactgtgcagggccacgtgtcgctccaggagggtcttgtgagagaacttctttttgcagatgtagcactcgtaggacttctctccccggtggaggcgcatgtgcacgttgagggagctcttctgggtgaagcgcttgttgcagatactacactggtatgccctcactcctgtgtgtgtcaccatgtgcttgataaggtaatcctttaaggagaaggagcgccaacagatgctgcattggtggggcttctcacctgtgtgtacgaacatgtgcttgacgtagttctgtttggcggtgaaagtcttgttgcagagagtgcactcataaggctttttttcgccttgcccactggctgtgctgtggcctgcggatgaggccaggggctgtggcgctggcagctgtgcagtaaaggtcgacagaccgggctgggacactgtcacaaactgggtctgctggcctgccaggggctgtggcaggctgaagaggaaaggcttggggccactgcccgcgggctgggtagtgaagagggctggcaggtaggtgttgccagctgtgccaatgacctgcgtgttgctggtcaaggtcagaggcatcctcaggttgctggtgagggtttctgtctggcgtaagtagagctgggtacttggcaatggctgcccgatggacgtgttgaccgaaggctgttgtaggacgctcttgtcggagctgttgctgacagtgataacagtgctgtccatctccacttcattgcttctctccggagaggaagcacctgtttctagctggtttgtctgcggaccaccctcagcgggggcttctgcagcctgctcgggttgggtgggttcagcctggctgtcccgcgccgccccaggcccaaactgctgctccaccgagtcaggctcggtgcctatggaggagctgacgcccgagtcgaagctttcacctttgggctcactctcggtgccctcggcctggtctgtgtcttccgtgcactcctcggattcgttgcgttccaggatctgcaccctttgctgcccgtagtagtcgtaatcgtcctccatctcctgcttgatgtggatgttgcccactagggtctggatgcgcacaggccggggctgcttgcggcagtgcgtggtctcgggggtggtggacaggtagcgctccatctgctgcgagcgctcatggatgcgtgtgatccagctggggtcttccatgtggtggtcgcggggcaggccgagcgcagtctcgtggtggctgaccactgcgccgctgtaaaaagagcgctcgccgctgccattctgcatggagcacgcgtagagtgccgagtagatcctgtccacgctgtgctgtgggtggctctgcaggtagcccgactccgtgtcgctgctctggcctgacgtgcctgactcgggagtgccccgcggcgtgtcctggcccgagtcctggatccccgggaacacatcgcccacgttctgtgacacgatgcgcgtgcactcgtcgatgactgttttgatctgcaggatgctggcggccgtgaggatctgcagagcttccgactgcgagacccgtagcacgccgctgtacatgaagtcaatgagcttttgcactgactgcactgacaccaccgacgggatctcgatgtcgctgtagccaagcagcagtttgtcctggaagaaggggctgccggctgccagcacgcagcggtgtgcgcgcagcatgctcccgtggatgcgcaccgttacgtcacagaagtggccacggttgcgctgctcgttgagggtctcgagcacggaattgctgaagttgtgaaggttgatgctgtgaatgcgctcggtcatccccttgcaactgatgtcacaatcagatgacccggtgtgagcgtgagagtttgtcagtgaatgtgttgagtggatgagggctgggtctggagacaaaacagcttcaaagttcaggcagggaaggcccggcttggcgctggatccacccggctgagtaatctcattctcctcagatgccttctggttttcagctgtcttgggtttcttcagtagtttcaaaatcaatggtgtcactcttcaggtaaattactccaaggcttgggcctagtgcagatgttcattggggcagggagcagagagcggctgcatgtaaagagaaggggcaggtcacagactgatggtcaaagatcagacagcaatgtcatgaggaatatcctgttagtaatgatgaaacattctgcacaagtctgaaacatcagtctatgtattttttttgaaatgtactctgtaccgatgcatttttctgtgtttctttctaaccctcgagaatgttaagaatttaggaagagagccacagcttaagagtgcaattatttgccagtaaatactcaatttgcttgtcctgtgatttttcttctaacttgcatattcaataatccgtccctgact

SEQ ID NO: 16688 - RNA, 12903 nt, Homo sapiens
  source 1..12903: mol_type = other RNA
taaaacccacaattatgtttgtctagtagaaatatatctgctggaacactttggagaacagattggtaattttgccattacactagacattagccctttcaaagcagactaagagtacgtagttccttagtgaatacaaggcttcacaactgaagagcattgcagggagcttggctaaggtgaaaagggacttgctggagaggtacagcagaatgggatgggattagaaaacaacaatctattaggaaagatgaaaggaaggaattccccagtgttcacgctgagaagtcttcatattggaccagtgtgagggggtcttttatactgaggttttaaaaacctgacttcattttgtcctgaatgtagaagtgaagaaggacactagtttcaggcacctgggatggtggaaaagtttattcaactgaggctttccatgcattgggttgaatagctgagggaagctgaagactcttatctgaaaatatgatctgaaaatatttattgtataggaagacagaatgcctgatttctgaagttttcttgatggcccaactaaagaagaaaggcaccaaatcctcactttaacaggtaaatggagatcctgagggctggatacccaagagccaccattttacggattcctcagatttaaaaatgtctcagatagatatttccaaattctatttctattagcctctgtggataaagagttcctgaaactctggttttactttttttggaaaaaaaaaaaaaaaaaaaaaaaaaaaacaactcccaggaaaatgaacactatattgccaagctgcctccagggaaaggttgaagactagttaaaataattctaagcgtattgaaaaaagaaagtgtaaagatccagtattaaaatgaatgtttgagaatacagtggggacaactaggtaattcactgtcttacgcttttcagaagactggccctttgaaacgcagcctgttattgttggtcagatcatgtggcacttaagtagccccttggtcatatttttaaaagcaaatatagacagtgacagtcctacaggggaaaatcacagatacattcatatgcacctcttttgttcttcagatattgagtgggtcagctaaacaagatcactttgaatatgaacctctttgtattagtcacaccaacaaaaaagtttcaaaaaaagttttcactttcctacatttgctaagtctgagctttaaaaaattctaaaatcctctaaagacaatactgaagctgataatataaaaagcaaattagagcactaatgattattactagatgcaccagattaactgcagcaggttggtgatgggtgatataagcaaagacataatatttcaatcaactcatgatcataggcagattcaaaagttaaaatgaatataatgtaatatatatttcaatatagagttgttatatataatgtgtatgtcctaggtttcagaaatactgcaatgtagtgtattgtagttaagtaagcatacctaaatagtaactcatattctttcacaaagtcactagtactgttaattaaaggaaaaaataaaaccgaaacaactaattgtttttccagtaaaaagaaatacctatggttacagttacagacttcttttggatatagaaagacaatatacattttaaaaagtaataacgacaaaaaagttgcaactgtaagtagccttacttaacaggggaaggggaaaagtcaccagaatagaagaggaaagaaaatgtcctctgacttctgtaaaacagaaataatgtacaaatcataaaaaataacaaaccatctagtaaaagaagggcatgggagtgagaaaactgaatcctgaattccaggccaccaaaccctcagagtccattcattcagtatattatactagagtggcattctacttcaatgcttgagatgggcaagagcaatcaattcctacagattaccaaaaaacattccccccaacagtctattggtttgctagacatggtaaacaacccactcctggaaagactttggcaaaggccacattggtttcaggagacacagtttgtgaattacgatgatatcttgtgagtacaggcagaattaggaagctttagtttgagaataaaatttatgtgtgtgtgtgtgtgtgtgtgtgtgtgtgtgcacactgcattgcatagaggaaaggaatgaagacctttgagctatgggatggctcaggccaaagtttgtgtgggctttgcctgcctggcattggtccccacccctgccacctccaggagacctggggagacgccctggactgctgctccctcttgtctgctcaccagttgaagacttctgttataccttattatggaggaaaacagcctgtccctgtgggtttgctgtggattcaacaagctgcatttgtttctcccaattctgaaacattacaaaaagcaacagagtgggcaggtgactgcttcctgggaagggagccacaagtcttaaacacaatggtgggaagaggcaactgtatctatgcacgaggacctctgcctgtgtgtgcttcctttggggggcacacacacttccagatgacaataagtatatacacaaacacacacatgtgcacacatgtcaataaatccaatagaactgtagagtttgttaaatgcactctactccacataagcatattcaagtttctcatgaaacggatacatagaaattactgatggttgggctccttcagaatgccctaaagtctcatcacagatactgatgcacccaactaaggcaacaaagcataagcagatacgtgagatatgtcagaccttcgacttctaaccagaagttcaaaaatgtatcttgttgtcactgggcaatatgaatgtgaaacagttttgtgctgagggaagctcacactgtgtgtgcacatgtataaataatgtatactcatttatagacattttggacagcagcggtgacatactggatgggttaagactctttcattattagaatctacatataaattgcaatgagtttgctgggtaaaaacaactgttgcaacactagtagaaacagatgcccccaaggtttttttttttttttttttttttttctctcttggatgtatcaaaatctcattgaggcattctaaaccaaagaaacctctgaatttgaaacagggttagtagggacttttatacccagctgggcatcccagaagcctggactctcaggactgtggctagattttgcccatgatctgtagattatgctcttgcaccggagacttgaaagttatgagtttgcattcaaacaaagaaccaccagataaaacagatgttctctaaaactgaggaaaaaaagtttagagatatacactgtatagagaaagaaagctttttgctggattgttctccttgttaaggaaatgtttaaaactagtactcccgggcacctgtgattgcattttataggattctatttagtaatatgatgtctattttacattcagccccaacctacgtcactgaaatagaataggaaatagcagccactatctgagagtacccagttctaggaaagtttggtgcctcctcaagaagtcactatttccatagtcctcaatcatgaatagggcttgtttttgtgataatgtaactattaaacagcaagaaatgcctataacttcagagccttctcatttctatatcttttatcctcttcccagggctttctgatttaaggcaataatgctacactataagtagccttttgtgaaaataccttaattgaggtcacttaagattagatttcagtctgaaagtctacagtttacggagcaaaaggtggagcctaaagaaaccactggcaggtgttttagtcagtggtgtggaaagataatgtttcttgtttcaacccagggcatttttacccatcatgcagtgaggagaaaatacatagttctgaaaaagaacccacactaggtagccctaattttctatctcttcactctaaaaaggatggaaacaagccctactgttccataaccattcccagggatcggctaaggtacattgctgactgctatagactcagtgttcaaggagaaaaaaatcttcagagacttagaaaactctttgcaatattttggtcaggctgatcgtcttgatactcagtgctagaaatgatgctttggattagtagtttccacattctgaatttataggaacactgagtcaccacagccttttttcttgtaaaggtttaagtgatatcagaaatagcaactctacacggaaagcccttgggaatatgaaaatactctctctcaagagcaagggctcttccgtgccccttttctgcctctgtatgtagcctgagcaccagggtagagattgcttttgaaagtttgccccatgtaatctatttcctggctacctaagagaacagccgttttcttcatgaaaacacaaagaggggaaagaggctgctgctgttccagtgggaagttatgtctagccccagaaggcctggtggctgggtcagctcaagcactctcttcatgcactgcaggctcaggaggcattgggttgctttgctttttctatggaattagggagcctattgaaattctagtgcacccctccttttgtttgtcaccaagtcacatggttctgtcttcagtatcctatttttctttttttttaatttctttttctgaggaacaaaattggccatttaaataaagttcttttctagtgagtaaagaggtttctcagagccagaaatcactgaaaagagagtctgtcgaccctgcccatggaaaagcccagagatttctctaaccacttcttgccaaacttcctagttttgtgattggatgtttcttggtttagcattgtttggtgctgaatacattttgcaattcttttgttctctgccctagagcttccattaccctggacttcaactcattaccaaattaaagaattcttttagaagatttcttttaagagtcaggtcacaacagaaagggcgccctcctgttctcctaaatctcaagggcatctcaggttgtgtctgctcttacgttgcaccttccttttgttcccttttaatgcagcagcacactggctatagcagaggcagacctgatttgattatctgataccttttccacaaaatcatatatcccctgctcccagccccaactaatcaaataacatcttctagaacaacagaggaaagctccagaatgggtgtatatcctgtgactcctggccagatccaccttgctccctgtcttcctaggggtcacaggtgttgggagcattgtggaggagccccaacaaggaagcaacatatggctttattatgttttctcaggaatcgaaggggttttataaggggcatatctcatttttgacttctgtgctgagagaaaatattgagttttgggcgcaggcagagcacagacaggacagctggtgttcctgtgtgagggaagtacacatagctcaaggctttaggactgaatgtgaaacaaacatacctggaggaaaacttttttcattatcagaattcacaaattcttactgttcatgggttgaaaaagagtatttgggaccttatagaatattttgatgatacaaaataaaacccttatgacttttaaacacagcaaacccaagtctttctaaggccaagagctactatgatctctaagatgactaggaatgaactgaggctagaatatgagcaggaaattatccagcacacttaatcatggcacaaatagattcaaagcattaggaatttgggaagagaacggtctataaaactgttattaggagctaaagtttacctctcaattaaaagatacaggaaaccattttgatacagagattttcatttcagattttttttctttgcttagcttgtttccccctgtgtagaattgtaacagatccatgtgttccaattattttcttttttaggattatatttcacacatttgggggccttttttgtacaaatattggcatgtaataaggaaaaattgcccatgatgctgagataataccagtgtttttagtggtagaaaatattatttttttataaaccatatctaaatatcttgagataaaaattcccctttgactttttttcctctcccttgtttggcaaattccattttaaaattataaattgctaaaaaatgtcctttccatactatttctctcttccttgtactcatcctaagaagtcttaaatctggaacatttgcttttatcttatctatctgtttcctggctactagaaagaaatttttttagcactcatatcaccctaccatgaaggtctaaatgtaagatgactgtaggacttgaaacaaaaaaaaattaaaaagatccacactcattctttgattttgaagcaaatgtctttccctatttctaaagatatttgtgattgtttaacttaaaagtgagaattgacaatctaaaagcatctctatccttttgaaacaggtccagattggtttatttcctaaaatgtgggtcagtttggaaagtggccatttgatgggccaggaacatagcaataaacaactacctctttgctcctccagattagatctcccactccaatccagcttcttcctctttccacaaaataatttgtcaactattttagaatgtgacatatttgggaaggataaatgtacagtaggaatatgtctactgctatgcaaacctggctggtccattttgtcatggactacaatgattatatcacctcattaagaattctttagggatcctccacctcctcccccactcccttttttttaagagacacttcctttacagggaaaggatgatagactcctcagggtttcaagtcacctgcagctttttctctacatgttctaccaaaagaaaaggtggattctaacccaattgcttagcattttacatggcaaatcagcattaaggcaaatgggtctctctcagatttgagaaacagaaagctacacgtggcccataatggcacctaagatcaacttttcaggcggtattagtgaaaattcttcctactttgctaaatttgaacaaagacactttcaaatctactgtgaaacagtttaaaatattttaaagtggcttttggccttctttcatttgtaacatgtattgagtgatttcatgtcattgtctcctagctttaagagtttttttcttaaggtcaatcttctcttttcattttatgggtggaatcacttgttttccaaaatatcaaaacaattccatgacatagttaattaatgctccctctattggtggtaagtggaaatattagtcttacaacactgctattttaaaaagcaaaattagcaatagaaaaatgaacttactttatctcggaagctgttcctcactaactgttaaaacagatcagttttggacatacagttcttggcaggactcctcttagaaatcacaataggttacacttaatagtcagttaaccacccaagtttacattaaaacttctagcaaaatatccactgaattaagcactgtgggaccaaatcaaactcacaaacacttcagttacactaaccttacaaagcatcacaaagaacttatgaaaaagatccaagttaaccaaatgtctaaaatatatgaataaaaccaatttagtcattacagagttgtttgtgttggaagattttccctcgtttgctgcacagtttttgtaaataaaatgctgacaggaaaattagaaggaaaattaaattaaaatgtaatgtaattttgaaactaaaatacgctctcctttcttctttttaaaactgtagtttggtgttttgctttgtttaaagatttgctttcccctaagtatgttaaaatatgcccagcaatgaaatcactttgggagtttcagctaggtttaagaattcctatatttgagctggaatcccttcaggacactgtctataatgaaaatgtctctattataacaccttgatcaggaccgaggagagaaatccctactaggaagagagagtggcatctggtatgatgcaatagattggtggtcttttgaatggtggctgttggcatctgggaatttttttgttaatttccctaaaacctttcgaagaagcaagggttaattcgtcatctaaagaatgatcatcttattcagccctcttaaccatggtggaaacagtcagaaggtgatatttggaaggaaaaaagtaattttggcatcaatgcatcttgatctataacaggcttctcataatgatgctctttgtagttgggaagggtgaggagctatggcagagttttgtgaactcctcttcctggctgatcacaaaagaaaagaccccatttatcaagacttctagactattagtgtttcactaagaaaaaaagtaaagtcaatagaaattctagaattgtaagatctcaatgaaattttggagaagcaagcaatctctttctgaaagataaagtctcttccatgaaaaagaacagaattctagatgaatcagttgaaaaaattattcagtggggcaacttaagcttgctaaagtcaaagaactacatatcaaaatacaaagcagcaattcaaattacagcagggatgggctggccacagaggccctcatcaacccaggcaatacttaaaataataaaaattaagaaaaattaaaaaaaatatgaagaaaatatccttcctctctttcaaatataactttagttgccttttattctttctatctggaagcagtatcgctaaccttaacagtcttgacttaccaaaaaatatatatatgtgtgtgaaataaaataaaagagaaggaattggtggcagtgtatgcaaaaccaaaatgaaaaaaattacttttaacaatttcactttttttgtttttttttttacacaaatactgttgtaaatatattaaaaaaatcagcattctatctggtaaacgtcacttttgcccctctataaaattttgaattaaaaaagcctcaagaactttttattgttccccccaccctccatttctttttctttttctcttccacaagaatatatcctgacactttttttttttttgcaaagattgttggaaataatccttctcttgtacctagaaacataggtgcaaatttctgatatctttgttttatctgcattcctgcctttcatgaaagtccctcttgattgtgctgaggctgtggctcagcgaagacactgaataaatacgatagccactgttgcttgttgcttgtccaagtcttcctggcttctgctgcaagagggggatatggagaaggtgggccagggtgtgtggacccgggcagaatctggggaagaagcctgccattcgtctttctttcccacaccaccgaacccactgcccttcccacccccacagcccttttatgaaatcagacaacgtggtaggtggaaaacagcagggcctttcctctgggttttcaaccagaagtgatattccacagttttaactggttactgtgaagtccaagcggccagaattgtgaaaatgtccactgaaacactgcaagcggtgtacttaaagacagtaggccttttagattttgttatatattttttgtagtgctcttcacaagtggaaattttttttttttttttacttttttttaaaagatttttttgtaaagaagggttgtatttagaggccagtagctagagatccaaccagtggacctcttgaagcactaccaggccttaaggccaccatccgagggagactgggaaaactattattcacccaagcctccggaaatgtaatgtaccagcaggcaaaaaacagttcttcatgtagtacaaaatgaaacgaaacaaaaacaaaaacagaaagtaaaaatgaaaccaaaacatttcttaaattctagtgccatagcttttttgtttgtttgttttttgttgttgttttgttttgttcataagaaagagagaaagatactacttatccgtcagacacatgcatcctcatgtggtcgttgaactgctcgatttggtcaaactttgctgggcagacggagcagacgtaagtggtcccctccgtgcaggccaccacgcctggggggccagcgcgggcacctgggggtgtgcctgcagggggggtcccattgctggcactgtgcagggccacgtgtcgctccaggagggtcttgtgagagaacttctttttgcagatgtagcactcgtaggacttctctccccggtggaggcgcatgtgcacgttgagggagctcttctgggtgaagcgcttgttgcagatactacactggtatgccctcactcctgtgtgtgtcaccatgtgcttgataaggtaatcctttaaggagaaggagcgccaacagatgctgcattggtggggcttctcacctgtgtgtacgaacatgtgcttgacgtagttctgtttggcggtgaaagtcttgttgcagagagtgcactcataaggctttttttcgccttgcccactggctgtgctgtggcctgcggatgaggccaggggctgtggcgctggcagctgtgcagtaaaggtcgacagaccgggctgggacactgtcacaaactgggtctgctggcctgccaggggctgtggcaggctgaagaggaaaggcttggggccactgcccgcgggctgggtagtgaagagggctggcaggtaggtgttgccagctgtgccaatgacctgcgtgttgctggtcaaggtcagaggcatcctcaggttgctggtgagggtttctgtctggcgtaagtagagctgggtacttggcaatggctgcccgatggacgtgttgaccgaaggctgttgtaggacgctcttgtcggagctgttgctgacagtgataacagtgctgtccatctccacttcattgcttctctccggagaggaagcacctgtttctagctggtttgtctgcggaccaccctcagcgggggcttctgcagcctgctcgggttgggtgggttcagcctggctgtcccgcgccgccccaggcccaaactgctgctccaccgagtcaggctcggtgcctatggaggagctgacgcccgagtcgaagctttcacctttgggctcactctcggtgccctcggcctggtctgtgtcttccgtgcactcctcggattcgttgcgttccaggatctgcaccctttgctgcccgtagtagtcgtaatcgtcctccatctcctgcttgatgtggatgttgcccactagggtctggatgcgcacaggccggggctgcttgcggcagtgcgtggtctcgggggtggtggacaggtagcgctccatctgctgcgagcgctcatggatgcgtgtgatccagctggggtcttccatgtggtggtcgcggggcaggccgagcgcagtctcgtggtggctgaccactgcgccgctgtaaaaagagcgctcgccgctgccattctgcatggagcacgcgtagagtgccgagtagatcctgtccacgctgtgctgtgggtggctctgcaggtagcccgactccgtgtcgctgctctggcctgacgtgcctgactcgggagtgccccgcggcgtgtcctggcccgagtcctggatccccgggaacacatcgcccacgttctgtgacacgatgcgcgtgcactcgtcgatgactgttttgatctgcaggatgctggcggccgtgaggatctgcagagcttccgactgcgagacccgtagcacgccgctgtacatgaagtcaatgagcttttgcactgactgcactgacaccaccgacgggatctcgatgtcgctgtagccaagcagcagtttgtcctggaagaaggggctgccggctgccagcacgcagcggtgtgcgcgcagcatgctcccgtggatgcgcaccgttacgtcacagaagtggccacggttgcgctgctcgttgagggtctcgagcacggaattgctgaagttgtgaaggttgatgctgtgaatgcgctcggtcatccccttgcaactgatgtcacaatcagatgacccggtgtgagcgtgagagtttgtcagtgaatgtgttgagtggatgagggctgggtctggagacaaaacagcttcaaagttcaggcagggaaggcccggcttggcgctggatccacccggctgagtaatctcattctcctcagatgccttctggttttcagctgtcttgggtttcttcagtagtttcaaaatcaatggtgtcactcttcaggtaaattactccaaggcttgggcctagtgcagatgttcattggggcagggagcagagagcggctgcatgtaaagagaaggggcaggtcacagactgatggtcaaagatcagacagcaatgtcatgaggaatatcctgttagtaatgatgaaacattctgtgaaataggtaataggaagccttggtaggtgctttcccaaacattgcaaataattctgaccacctccagctgactctgatgtatccacctccatggggttgttgtcattatttggacatttccagaaatcaagatccacttcagtttgtgaagatgagctgtgcttagacataggctgtgcagctatggggcacaaacttgcaattcatcaattcttcagccttcagagtcccaaaggcaattcttaacacttctttttatttgtagtggcatggatgacggagcagaaatagagaattcttgattaaccaggagaagaatatcataggcatgggtgtgagatcaactggagattcaaggaagctaaagtgcccagaatgaactaatgttgtaatgtagactgtgagcagagataaaattccagaagccaaggagtgttgtacggtaagtcctggcagtgc

SEQ ID NO: 16689 - RNA, 12482 nt, Homo sapiens
  source 1..12482: mol_type = other RNA
taaaacccacaattatgtttgtctagtagaaatatatctgctggaacactttggagaacagattggtaattttgccattacactagacattagccctttcaaagcagactaagagtacgtagttccttagtgaatacaaggcttcacaactgaagagcattgcagggagcttggctaaggtgaaaagggacttgctggagaggtacagcagaatgggatgggattagaaaacaacaatctattaggaaagatgaaaggaaggaattccccagtgttcacgctgagaagtcttcatattggaccagtgtgagggggtcttttatactgaggttttaaaaacctgacttcattttgtcctgaatgtagaagtgaagaaggacactagtttcaggcacctgggatggtggaaaagtttattcaactgaggctttccatgcattgggttgaatagctgagggaagctgaagactcttatctgaaaatatgatctgaaaatatttattgtataggaagacagaatgcctgatttctgaagttttcttgatggcccaactaaagaagaaaggcaccaaatcctcactttaacaggtaaatggagatcctgagggctggatacccaagagccaccattttacggattcctcagatttaaaaatgtctcagatagatatttccaaattctatttctattagcctctgtggataaagagttcctgaaactctggttttactttttttggaaaaaaaaaaaaaaaaaaaaaaaaaaaacaactcccaggaaaatgaacactatattgccaagctgcctccagggaaaggttgaagactagttaaaataattctaagcgtattgaaaaaagaaagtgtaaagatccagtattaaaatgaatgtttgagaatacagtggggacaactaggtaattcactgtcttacgcttttcagaagactggccctttgaaacgcagcctgttattgttggtcagatcatgtggcacttaagtagccccttggtcatatttttaaaagcaaatatagacagtgacagtcctacaggggaaaatcacagatacattcatatgcacctcttttgttcttcagatattgagtgggtcagctaaacaagatcactttgaatatgaacctctttgtattagtcacaccaacaaaaaagtttcaaaaaaagttttcactttcctacatttgctaagtctgagctttaaaaaattctaaaatcctctaaagacaatactgaagctgataatataaaaagcaaattagagcactaatgattattactagatgcaccagattaactgcagcaggttggtgatgggtgatataagcaaagacataatatttcaatcaactcatgatcataggcagattcaaaagttaaaatgaatataatgtaatatatatttcaatatagagttgttatatataatgtgtatgtcctaggtttcagaaatactgcaatgtagtgtattgtagttaagtaagcatacctaaatagtaactcatattctttcacaaagtcactagtactgttaattaaaggaaaaaataaaaccgaaacaactaattgtttttccagtaaaaagaaatacctatggttacagttacagacttcttttggatatagaaagacaatatacattttaaaaagtaataacgacaaaaaagttgcaactgtaagtagccttacttaacaggggaaggggaaaagtcaccagaatagaagaggaaagaaaatgtcctctgacttctgtaaaacagaaataatgtacaaatcataaaaaataacaaaccatctagtaaaagaagggcatgggagtgagaaaactgaatcctgaattccaggccaccaaaccctcagagtccattcattcagtatattatactagagtggcattctacttcaatgcttgagatgggcaagagcaatcaattcctacagattaccaaaaaacattccccccaacagtctattggtttgctagacatggtaaacaacccactcctggaaagactttggcaaaggccacattggtttcaggagacacagtttgtgaattacgatgatatcttgtgagtacaggcagaattaggaagctttagtttgagaataaaatttatgtgtgtgtgtgtgtgtgtgtgtgtgtgtgtgcacactgcattgcatagaggaaaggaatgaagacctttgagctatgggatggctcaggccaaagtttgtgtgggctttgcctgcctggcattggtccccacccctgccacctccaggagacctggggagacgccctggactgctgctccctcttgtctgctcaccagttgaagacttctgttataccttattatggaggaaaacagcctgtccctgtgggtttgctgtggattcaacaagctgcatttgtttctcccaattctgaaacattacaaaaagcaacagagtgggcaggtgactgcttcctgggaagggagccacaagtcttaaacacaatggtgggaagaggcaactgtatctatgcacgaggacctctgcctgtgtgtgcttcctttggggggcacacacacttccagatgacaataagtatatacacaaacacacacatgtgcacacatgtcaataaatccaatagaactgtagagtttgttaaatgcactctactccacataagcatattcaagtttctcatgaaacggatacatagaaattactgatggttgggctccttcagaatgccctaaagtctcatcacagatactgatgcacccaactaaggcaacaaagcataagcagatacgtgagatatgtcagaccttcgacttctaaccagaagttcaaaaatgtatcttgttgtcactgggcaatatgaatgtgaaacagttttgtgctgagggaagctcacactgtgtgtgcacatgtataaataatgtatactcatttatagacattttggacagcagcggtgacatactggatgggttaagactctttcattattagaatctacatataaattgcaatgagtttgctgggtaaaaacaactgttgcaacactagtagaaacagatgcccccaaggtttttttttttttttttttttttttctctcttggatgtatcaaaatctcattgaggcattctaaaccaaagaaacctctgaatttgaaacagggttagtagggacttttatacccagctgggcatcccagaagcctggactctcaggactgtggctagattttgcccatgatctgtagattatgctcttgcaccggagacttgaaagttatgagtttgcattcaaacaaagaaccaccagataaaacagatgttctctaaaactgaggaaaaaaagtttagagatatacactgtatagagaaagaaagctttttgctggattgttctccttgttaaggaaatgtttaaaactagtactcccgggcacctgtgattgcattttataggattctatttagtaatatgatgtctattttacattcagccccaacctacgtcactgaaatagaataggaaatagcagccactatctgagagtacccagttctaggaaagtttggtgcctcctcaagaagtcactatttccatagtcctcaatcatgaatagggcttgtttttgtgataatgtaactattaaacagcaagaaatgcctataacttcagagccttctcatttctatatcttttatcctcttcccagggctttctgatttaaggcaataatgctacactataagtagccttttgtgaaaataccttaattgaggtcacttaagattagatttcagtctgaaagtctacagtttacggagcaaaaggtggagcctaaagaaaccactggcaggtgttttagtcagtggtgtggaaagataatgtttcttgtttcaacccagggcatttttacccatcatgcagtgaggagaaaatacatagttctgaaaaagaacccacactaggtagccctaattttctatctcttcactctaaaaaggatggaaacaagccctactgttccataaccattcccagggatcggctaaggtacattgctgactgctatagactcagtgttcaaggagaaaaaaatcttcagagacttagaaaactctttgcaatattttggtcaggctgatcgtcttgatactcagtgctagaaatgatgctttggattagtagtttccacattctgaatttataggaacactgagtcaccacagccttttttcttgtaaaggtttaagtgatatcagaaatagcaactctacacggaaagcccttgggaatatgaaaatactctctctcaagagcaagggctcttccgtgccccttttctgcctctgtatgtagcctgagcaccagggtagagattgcttttgaaagtttgccccatgtaatctatttcctggctacctaagagaacagccgttttcttcatgaaaacacaaagaggggaaagaggctgctgctgttccagtgggaagttatgtctagccccagaaggcctggtggctgggtcagctcaagcactctcttcatgcactgcaggctcaggaggcattgggttgctttgctttttctatggaattagggagcctattgaaattctagtgcacccctccttttgtttgtcaccaagtcacatggttctgtcttcagtatcctatttttctttttttttaatttctttttctgaggaacaaaattggccatttaaataaagttcttttctagtgagtaaagaggtttctcagagccagaaatcactgaaaagagagtctgtcgaccctgcccatggaaaagcccagagatttctctaaccacttcttgccaaacttcctagttttgtgattggatgtttcttggtttagcattgtttggtgctgaatacattttgcaattcttttgttctctgccctagagcttccattaccctggacttcaactcattaccaaattaaagaattcttttagaagatttcttttaagagtcaggtcacaacagaaagggcgccctcctgttctcctaaatctcaagggcatctcaggttgtgtctgctcttacgttgcaccttccttttgttcccttttaatgcagcagcacactggctatagcagaggcagacctgatttgattatctgataccttttccacaaaatcatatatcccctgctcccagccccaactaatcaaataacatcttctagaacaacagaggaaagctccagaatgggtgtatatcctgtgactcctggccagatccaccttgctccctgtcttcctaggggtcacaggtgttgggagcattgtggaggagccccaacaaggaagcaacatatggctttattatgttttctcaggaatcgaaggggttttataaggggcatatctcatttttgacttctgtgctgagagaaaatattgagttttgggcgcaggcagagcacagacaggacagctggtgttcctgtgtgagggaagtacacatagctcaaggctttaggactgaatgtgaaacaaacatacctggaggaaaacttttttcattatcagaattcacaaattcttactgttcatgggttgaaaaagagtatttgggaccttatagaatattttgatgatacaaaataaaacccttatgacttttaaacacagcaaacccaagtctttctaaggccaagagctactatgatctctaagatgactaggaatgaactgaggctagaatatgagcaggaaattatccagcacacttaatcatggcacaaatagattcaaagcattaggaatttgggaagagaacggtctataaaactgttattaggagctaaagtttacctctcaattaaaagatacaggaaaccattttgatacagagattttcatttcagattttttttctttgcttagcttgtttccccctgtgtagaattgtaacagatccatgtgttccaattattttcttttttaggattatatttcacacatttgggggccttttttgtacaaatattggcatgtaataaggaaaaattgcccatgatgctgagataataccagtgtttttagtggtagaaaatattatttttttataaaccatatctaaatatcttgagataaaaattcccctttgactttttttcctctcccttgtttggcaaattccattttaaaattataaattgctaaaaaatgtcctttccatactatttctctcttccttgtactcatcctaagaagtcttaaatctggaacatttgcttttatcttatctatctgtttcctggctactagaaagaaatttttttagcactcatatcaccctaccatgaaggtctaaatgtaagatgactgtaggacttgaaacaaaaaaaaattaaaaagatccacactcattctttgattttgaagcaaatgtctttccctatttctaaagatatttgtgattgtttaacttaaaagtgagaattgacaatctaaaagcatctctatccttttgaaacaggtccagattggtttatttcctaaaatgtgggtcagtttggaaagtggccatttgatgggccaggaacatagcaataaacaactacctctttgctcctccagattagatctcccactccaatccagcttcttcctctttccacaaaataatttgtcaactattttagaatgtgacatatttgggaaggataaatgtacagtaggaatatgtctactgctatgcaaacctggctggtccattttgtcatggactacaatgattatatcacctcattaagaattctttagggatcctccacctcctcccccactcccttttttttaagagacacttcctttacagggaaaggatgatagactcctcagggtttcaagtcacctgcagctttttctctacatgttctaccaaaagaaaaggtggattctaacccaattgcttagcattttacatggcaaatcagcattaaggcaaatgggtctctctcagatttgagaaacagaaagctacacgtggcccataatggcacctaagatcaacttttcaggcggtattagtgaaaattcttcctactttgctaaatttgaacaaagacactttcaaatctactgtgaaacagtttaaaatattttaaagtggcttttggccttctttcatttgtaacatgtattgagtgatttcatgtcattgtctcctagctttaagagtttttttcttaaggtcaatcttctcttttcattttatgggtggaatcacttgttttccaaaatatcaaaacaattccatgacatagttaattaatgctccctctattggtggtaagtggaaatattagtcttacaacactgctattttaaaaagcaaaattagcaatagaaaaatgaacttactttatctcggaagctgttcctcactaactgttaaaacagatcagttttggacatacagttcttggcaggactcctcttagaaatcacaataggttacacttaatagtcagttaaccacccaagtttacattaaaacttctagcaaaatatccactgaattaagcactgtgggaccaaatcaaactcacaaacacttcagttacactaaccttacaaagcatcacaaagaacttatgaaaaagatccaagttaaccaaatgtctaaaatatatgaataaaaccaatttagtcattacagagttgtttgtgttggaagattttccctcgtttgctgcacagtttttgtaaataaaatgctgacaggaaaattagaaggaaaattaaattaaaatgtaatgtaattttgaaactaaaatacgctctcctttcttctttttaaaactgtagtttggtgttttgctttgtttaaagatttgctttcccctaagtatgttaaaatatgcccagcaatgaaatcactttgggagtttcagctaggtttaagaattcctatatttgagctggaatcccttcaggacactgtctataatgaaaatgtctctattataacaccttgatcaggaccgaggagagaaatccctactaggaagagagagtggcatctggtatgatgcaatagattggtggtcttttgaatggtggctgttggcatctgggaatttttttgttaatttccctaaaacctttcgaagaagcaagggttaattcgtcatctaaagaatgatcatcttattcagccctcttaaccatggtggaaacagtcagaaggtgatatttggaaggaaaaaagtaattttggcatcaatgcatcttgatctataacaggcttctcataatgatgctctttgtagttgggaagggtgaggagctatggcagagttttgtgaactcctcttcctggctgatcacaaaagaaaagaccccatttatcaagacttctagactattagtgtttcactaagaaaaaaagtaaagtcaatagaaattctagaattgtaagatctcaatgaaattttggagaagcaagcaatctctttctgaaagataaagtctcttccatgaaaaagaacagaattctagatgaatcagttgaaaaaattattcagtggggcaacttaagcttgctaaagtcaaagaactacatatcaaaatacaaagcagcaattcaaattacagcagggatgggctggccacagaggccctcatcaacccaggcaatacttaaaataataaaaattaagaaaaattaaaaaaaatatgaagaaaatatccttcctctctttcaaatataactttagttgccttttattctttctatctggaagcagtatcgctaaccttaacagtcttgacttaccaaaaaatatatatatgtgtgtgaaataaaataaaagagaaggaattggtggcagtgtatgcaaaaccaaaatgaaaaaaattacttttaacaatttcactttttttgtttttttttttacacaaatactgttgtaaatatattaaaaaaatcagcattctatctggtaaacgtcacttttgcccctctataaaattttgaattaaaaaagcctcaagaactttttattgttccccccaccctccatttctttttctttttctcttccacaagaatatatcctgacactttttttttttttgcaaagattgttggaaataatccttctcttgtacctagaaacataggtgcaaatttctgatatctttgttttatctgcattcctgcctttcatgaaagtccctcttgattgtgctgaggctgtggctcagcgaagacactgaataaatacgatagccactgttgcttgttgcttgtccaagtcttcctggcttctgctgcaagagggggatatggagaaggtgggccagggtgtgtggacccgggcagaatctggggaagaagcctgccattcgtctttctttcccacaccaccgaacccactgcccttcccacccccacagcccttttatgaaatcagacaacgtggtaggtggaaaacagcagggcctttcctctgggttttcaaccagaagtgatattccacagttttaactggttactgtgaagtccaagcggccagaattgtgaaaatgtccactgaaacactgcaagcggtgtacttaaagacagtaggccttttagattttgttatatattttttgtagtgctcttcacaagtggaaattttttttttttttttacttttttttaaaagatttttttgtaaagaagggttgtatttagaggccagtagctagagatccaaccagtggacctcttgaagcactaccaggccttaaggccaccatccgagggagactgggaaaactattattcacccaagcctccggaaatgtaatgtaccagcaggcaaaaaacagttcttcatgtagtacaaaatgaaacgaaacaaaaacaaaaacagaaagtaaaaatgaaaccaaaacatttcttaaattctagtgccatagcttttttgtttgtttgttttttgttgttgttttgttttgttcataagaaagagagaaagatactacttatccgtcagacacatgcatcctcatgtggtcgttgaactgctcgatttggtcaaactttgctgggcagacggagcagacgtaagtggtcccctccgtgcaggccaccacgcctggggggccagcgcgggcacctgggggtgtgcctgcagggggggtcccattgctggcactgtgcagggccacgtgtcgctccaggagggtcttgtgagagaacttctttttgcagatgtagcactcgtaggacttctctccccggtggaggcgcatgtgcacgttgagggagctcttctgggtgaagcgcttgttgcagatactacactggtatgccctcactcctgtgtgtgtcaccatgtgcttgataaggtaatcctttaaggagaaggagcgccaacagatgctgcattggtggggcttctcacctgtgtgtacgaacatgtgcttgacgtagttctgtttggcggtgaaagtcttgttgcagagagtgcactcataaggctttttttcgccttgcccactggctgtgctgtggcctgcggatgaggccaggggctgtggcgctggcagctgtgcagtaaaggtcgacagaccgggctgggacactgtcacaaactgggtctgctggcctgccaggggctgtggcaggctgaagaggaaaggcttggggccactgcccgcgggctgggtagtgaagagggctggcaggtaggtgttgccagctgtgccaatgacctgcgtgttgctggtcaaggtcagaggcatcctcaggttgctggtgagggtttctgtctggcgtaagtagagctgggtacttggcaatggctgcccgatggacgtgttgaccgaaggctgttgtaggacgctcttgtcggagctgttgctgacagtgataacagtgctgtccatctccacttcattgcttctctccggagaggaagcacctgtttctagctggtttgtctgcggaccaccctcagcgggggcttctgcagcctgctcgggttgggtgggttcagcctggctgtcccgcgccgccccaggcccaaactgctgctccaccgagtcaggctcggtgcctatggaggagctgacgcccgagtcgaagctttcacctttgggctcactctcggtgccctcggcctggtctgtgtcttccgtgcactcctcggattcgttgcgttccaggatctgcaccctttgctgcccgtagtagtcgtaatcgtcctccatctcctgcttgatgtggatgttgcccactagggtctggatgcgcacaggccggggctgcttgcggcagtgcgtggtctcgggggtggtggacaggtagcgctccatctgctgcgagcgctcatggatgcgtgtgatccagctggggtcttccatgtggtggtcgcggggcaggccgagcgcagtctcgtggtggctgaccactgcgccgctgtaaaaagagcgctcgccgctgccattctgcatggagcacgcgtagagtgccgagtagatcctgtccacgctgtgctgtgggtggctctgcaggtagcccgactccgtgtcgctgctctggcctgacgtgcctgactcgggagtgccccgcggcgtgtcctggcccgagtcctggatccccgggaacacatcgcccacgttctgtgacacgatgcgcgtgcactcgtcgatgactgttttgatctgcaggatgctggcggccgtgaggatctgcagagcttccgactgcgagacccgtagcacgccgctgtacatgaagtcaatgagcttttgcactgactgcactgacaccaccgacgggatctcgatgtcgctgtagccaagcagcagtttgtcctggaagaaggggctgccggctgccagcacgcagcggtgtgcgcgcagcatgctcccgtggatgcgcaccgttacgtcacagaagtggccacggttgcgctgctcgttgagggtctcgagcacggaattgctgaagttgtgaaggttgatgctgtgaatgcgctcggtcatccccttgcaactgatgtcacaatcagatgacccggtgtgagcgtgagagtttgtcagtgaatgtgttgagtggatgagggctgggtctggagacaaaacagcttcaaagttcaggcagggaaggcccggcttggcgctggatccacccggctgagtaatctcattctcctcagatgccttctggttttcagctgtcttgggtttcttcagtagtttcaaaatcaatggtgtcactcttcaggtaaattactccaaggcttgggcctagtgcagatgttcattggggcagggagcagagagcggctgcatgtaaagagaaggggcaggtcacagactgatggtcaaagatcaggactatggttcctgatccaaggagtgacgactgagaatcagcacacagtctcttgagggtgtccaggcctggctgttaagctccctgc

SEQ ID NO: 16690 - RNA, 12460 nt, Homo sapiens
  source 1..12460: mol_type = other RNA
taaaacccacaattatgtttgtctagtagaaatatatctgctggaacactttggagaacagattggtaattttgccattacactagacattagccctttcaaagcagactaagagtacgtagttccttagtgaatacaaggcttcacaactgaagagcattgcagggagcttggctaaggtgaaaagggacttgctggagaggtacagcagaatgggatgggattagaaaacaacaatctattaggaaagatgaaaggaaggaattccccagtgttcacgctgagaagtcttcatattggaccagtgtgagggggtcttttatactgaggttttaaaaacctgacttcattttgtcctgaatgtagaagtgaagaaggacactagtttcaggcacctgggatggtggaaaagtttattcaactgaggctttccatgcattgggttgaatagctgagggaagctgaagactcttatctgaaaatatgatctgaaaatatttattgtataggaagacagaatgcctgatttctgaagttttcttgatggcccaactaaagaagaaaggcaccaaatcctcactttaacaggtaaatggagatcctgagggctggatacccaagagccaccattttacggattcctcagatttaaaaatgtctcagatagatatttccaaattctatttctattagcctctgtggataaagagttcctgaaactctggttttactttttttggaaaaaaaaaaaaaaaaaaaaaaaaaaaacaactcccaggaaaatgaacactatattgccaagctgcctccagggaaaggttgaagactagttaaaataattctaagcgtattgaaaaaagaaagtgtaaagatccagtattaaaatgaatgtttgagaatacagtggggacaactaggtaattcactgtcttacgcttttcagaagactggccctttgaaacgcagcctgttattgttggtcagatcatgtggcacttaagtagccccttggtcatatttttaaaagcaaatatagacagtgacagtcctacaggggaaaatcacagatacattcatatgcacctcttttgttcttcagatattgagtgggtcagctaaacaagatcactttgaatatgaacctctttgtattagtcacaccaacaaaaaagtttcaaaaaaagttttcactttcctacatttgctaagtctgagctttaaaaaattctaaaatcctctaaagacaatactgaagctgataatataaaaagcaaattagagcactaatgattattactagatgcaccagattaactgcagcaggttggtgatgggtgatataagcaaagacataatatttcaatcaactcatgatcataggcagattcaaaagttaaaatgaatataatgtaatatatatttcaatatagagttgttatatataatgtgtatgtcctaggtttcagaaatactgcaatgtagtgtattgtagttaagtaagcatacctaaatagtaactcatattctttcacaaagtcactagtactgttaattaaaggaaaaaataaaaccgaaacaactaattgtttttccagtaaaaagaaatacctatggttacagttacagacttcttttggatatagaaagacaatatacattttaaaaagtaataacgacaaaaaagttgcaactgtaagtagccttacttaacaggggaaggggaaaagtcaccagaatagaagaggaaagaaaatgtcctctgacttctgtaaaacagaaataatgtacaaatcataaaaaataacaaaccatctagtaaaagaagggcatgggagtgagaaaactgaatcctgaattccaggccaccaaaccctcagagtccattcattcagtatattatactagagtggcattctacttcaatgcttgagatgggcaagagcaatcaattcctacagattaccaaaaaacattccccccaacagtctattggtttgctagacatggtaaacaacccactcctggaaagactttggcaaaggccacattggtttcaggagacacagtttgtgaattacgatgatatcttgtgagtacaggcagaattaggaagctttagtttgagaataaaatttatgtgtgtgtgtgtgtgtgtgtgtgtgtgtgtgcacactgcattgcatagaggaaaggaatgaagacctttgagctatgggatggctcaggccaaagtttgtgtgggctttgcctgcctggcattggtccccacccctgccacctccaggagacctggggagacgccctggactgctgctccctcttgtctgctcaccagttgaagacttctgttataccttattatggaggaaaacagcctgtccctgtgggtttgctgtggattcaacaagctgcatttgtttctcccaattctgaaacattacaaaaagcaacagagtgggcaggtgactgcttcctgggaagggagccacaagtcttaaacacaatggtgggaagaggcaactgtatctatgcacgaggacctctgcctgtgtgtgcttcctttggggggcacacacacttccagatgacaataagtatatacacaaacacacacatgtgcacacatgtcaataaatccaatagaactgtagagtttgttaaatgcactctactccacataagcatattcaagtttctcatgaaacggatacatagaaattactgatggttgggctccttcagaatgccctaaagtctcatcacagatactgatgcacccaactaaggcaacaaagcataagcagatacgtgagatatgtcagaccttcgacttctaaccagaagttcaaaaatgtatcttgttgtcactgggcaatatgaatgtgaaacagttttgtgctgagggaagctcacactgtgtgtgcacatgtataaataatgtatactcatttatagacattttggacagcagcggtgacatactggatgggttaagactctttcattattagaatctacatataaattgcaatgagtttgctgggtaaaaacaactgttgcaacactagtagaaacagatgcccccaaggtttttttttttttttttttttttttctctcttggatgtatcaaaatctcattgaggcattctaaaccaaagaaacctctgaatttgaaacagggttagtagggacttttatacccagctgggcatcccagaagcctggactctcaggactgtggctagattttgcccatgatctgtagattatgctcttgcaccggagacttgaaagttatgagtttgcattcaaacaaagaaccaccagataaaacagatgttctctaaaactgaggaaaaaaagtttagagatatacactgtatagagaaagaaagctttttgctggattgttctccttgttaaggaaatgtttaaaactagtactcccgggcacctgtgattgcattttataggattctatttagtaatatgatgtctattttacattcagccccaacctacgtcactgaaatagaataggaaatagcagccactatctgagagtacccagttctaggaaagtttggtgcctcctcaagaagtcactatttccatagtcctcaatcatgaatagggcttgtttttgtgataatgtaactattaaacagcaagaaatgcctataacttcagagccttctcatttctatatcttttatcctcttcccagggctttctgatttaaggcaataatgctacactataagtagccttttgtgaaaataccttaattgaggtcacttaagattagatttcagtctgaaagtctacagtttacggagcaaaaggtggagcctaaagaaaccactggcaggtgttttagtcagtggtgtggaaagataatgtttcttgtttcaacccagggcatttttacccatcatgcagtgaggagaaaatacatagttctgaaaaagaacccacactaggtagccctaattttctatctcttcactctaaaaaggatggaaacaagccctactgttccataaccattcccagggatcggctaaggtacattgctgactgctatagactcagtgttcaaggagaaaaaaatcttcagagacttagaaaactctttgcaatattttggtcaggctgatcgtcttgatactcagtgctagaaatgatgctttggattagtagtttccacattctgaatttataggaacactgagtcaccacagccttttttcttgtaaaggtttaagtgatatcagaaatagcaactctacacggaaagcccttgggaatatgaaaatactctctctcaagagcaagggctcttccgtgccccttttctgcctctgtatgtagcctgagcaccagggtagagattgcttttgaaagtttgccccatgtaatctatttcctggctacctaagagaacagccgttttcttcatgaaaacacaaagaggggaaagaggctgctgctgttccagtgggaagttatgtctagccccagaaggcctggtggctgggtcagctcaagcactctcttcatgcactgcaggctcaggaggcattgggttgctttgctttttctatggaattagggagcctattgaaattctagtgcacccctccttttgtttgtcaccaagtcacatggttctgtcttcagtatcctatttttctttttttttaatttctttttctgaggaacaaaattggccatttaaataaagttcttttctagtgagtaaagaggtttctcagagccagaaatcactgaaaagagagtctgtcgaccctgcccatggaaaagcccagagatttctctaaccacttcttgccaaacttcctagttttgtgattggatgtttcttggtttagcattgtttggtgctgaatacattttgcaattcttttgttctctgccctagagcttccattaccctggacttcaactcattaccaaattaaagaattcttttagaagatttcttttaagagtcaggtcacaacagaaagggcgccctcctgttctcctaaatctcaagggcatctcaggttgtgtctgctcttacgttgcaccttccttttgttcccttttaatgcagcagcacactggctatagcagaggcagacctgatttgattatctgataccttttccacaaaatcatatatcccctgctcccagccccaactaatcaaataacatcttctagaacaacagaggaaagctccagaatgggtgtatatcctgtgactcctggccagatccaccttgctccctgtcttcctaggggtcacaggtgttgggagcattgtggaggagccccaacaaggaagcaacatatggctttattatgttttctcaggaatcgaaggggttttataaggggcatatctcatttttgacttctgtgctgagagaaaatattgagttttgggcgcaggcagagcacagacaggacagctggtgttcctgtgtgagggaagtacacatagctcaaggctttaggactgaatgtgaaacaaacatacctggaggaaaacttttttcattatcagaattcacaaattcttactgttcatgggttgaaaaagagtatttgggaccttatagaatattttgatgatacaaaataaaacccttatgacttttaaacacagcaaacccaagtctttctaaggccaagagctactatgatctctaagatgactaggaatgaactgaggctagaatatgagcaggaaattatccagcacacttaatcatggcacaaatagattcaaagcattaggaatttgggaagagaacggtctataaaactgttattaggagctaaagtttacctctcaattaaaagatacaggaaaccattttgatacagagattttcatttcagattttttttctttgcttagcttgtttccccctgtgtagaattgtaacagatccatgtgttccaattattttcttttttaggattatatttcacacatttgggggccttttttgtacaaatattggcatgtaataaggaaaaattgcccatgatgctgagataataccagtgtttttagtggtagaaaatattatttttttataaaccatatctaaatatcttgagataaaaattcccctttgactttttttcctctcccttgtttggcaaattccattttaaaattataaattgctaaaaaatgtcctttccatactatttctctcttccttgtactcatcctaagaagtcttaaatctggaacatttgcttttatcttatctatctgtttcctggctactagaaagaaatttttttagcactcatatcaccctaccatgaaggtctaaatgtaagatgactgtaggacttgaaacaaaaaaaaattaaaaagatccacactcattctttgattttgaagcaaatgtctttccctatttctaaagatatttgtgattgtttaacttaaaagtgagaattgacaatctaaaagcatctctatccttttgaaacaggtccagattggtttatttcctaaaatgtgggtcagtttggaaagtggccatttgatgggccaggaacatagcaataaacaactacctctttgctcctccagattagatctcccactccaatccagcttcttcctctttccacaaaataatttgtcaactattttagaatgtgacatatttgggaaggataaatgtacagtaggaatatgtctactgctatgcaaacctggctggtccattttgtcatggactacaatgattatatcacctcattaagaattctttagggatcctccacctcctcccccactcccttttttttaagagacacttcctttacagggaaaggatgatagactcctcagggtttcaagtcacctgcagctttttctctacatgttctaccaaaagaaaaggtggattctaacccaattgcttagcattttacatggcaaatcagcattaaggcaaatgggtctctctcagatttgagaaacagaaagctacacgtggcccataatggcacctaagatcaacttttcaggcggtattagtgaaaattcttcctactttgctaaatttgaacaaagacactttcaaatctactgtgaaacagtttaaaatattttaaagtggcttttggccttctttcatttgtaacatgtattgagtgatttcatgtcattgtctcctagctttaagagtttttttcttaaggtcaatcttctcttttcattttatgggtggaatcacttgttttccaaaatatcaaaacaattccatgacatagttaattaatgctccctctattggtggtaagtggaaatattagtcttacaacactgctattttaaaaagcaaaattagcaatagaaaaatgaacttactttatctcggaagctgttcctcactaactgttaaaacagatcagttttggacatacagttcttggcaggactcctcttagaaatcacaataggttacacttaatagtcagttaaccacccaagtttacattaaaacttctagcaaaatatccactgaattaagcactgtgggaccaaatcaaactcacaaacacttcagttacactaaccttacaaagcatcacaaagaacttatgaaaaagatccaagttaaccaaatgtctaaaatatatgaataaaaccaatttagtcattacagagttgtttgtgttggaagattttccctcgtttgctgcacagtttttgtaaataaaatgctgacaggaaaattagaaggaaaattaaattaaaatgtaatgtaattttgaaactaaaatacgctctcctttcttctttttaaaactgtagtttggtgttttgctttgtttaaagatttgctttcccctaagtatgttaaaatatgcccagcaatgaaatcactttgggagtttcagctaggtttaagaattcctatatttgagctggaatcccttcaggacactgtctataatgaaaatgtctctattataacaccttgatcaggaccgaggagagaaatccctactaggaagagagagtggcatctggtatgatgcaatagattggtggtcttttgaatggtggctgttggcatctgggaatttttttgttaatttccctaaaacctttcgaagaagcaagggttaattcgtcatctaaagaatgatcatcttattcagccctcttaaccatggtggaaacagtcagaaggtgatatttggaaggaaaaaagtaattttggcatcaatgcatcttgatctataacaggcttctcataatgatgctctttgtagttgggaagggtgaggagctatggcagagttttgtgaactcctcttcctggctgatcacaaaagaaaagaccccatttatcaagacttctagactattagtgtttcactaagaaaaaaagtaaagtcaatagaaattctagaattgtaagatctcaatgaaattttggagaagcaagcaatctctttctgaaagataaagtctcttccatgaaaaagaacagaattctagatgaatcagttgaaaaaattattcagtggggcaacttaagcttgctaaagtcaaagaactacatatcaaaatacaaagcagcaattcaaattacagcagggatgggctggccacagaggccctcatcaacccaggcaatacttaaaataataaaaattaagaaaaattaaaaaaaatatgaagaaaatatccttcctctctttcaaatataactttagttgccttttattctttctatctggaagcagtatcgctaaccttaacagtcttgacttaccaaaaaatatatatatgtgtgtgaaataaaataaaagagaaggaattggtggcagtgtatgcaaaaccaaaatgaaaaaaattacttttaacaatttcactttttttgtttttttttttacacaaatactgttgtaaatatattaaaaaaatcagcattctatctggtaaacgtcacttttgcccctctataaaattttgaattaaaaaagcctcaagaactttttattgttccccccaccctccatttctttttctttttctcttccacaagaatatatcctgacactttttttttttttgcaaagattgttggaaataatccttctcttgtacctagaaacataggtgcaaatttctgatatctttgttttatctgcattcctgcctttcatgaaagtccctcttgattgtgctgaggctgtggctcagcgaagacactgaataaatacgatagccactgttgcttgttgcttgtccaagtcttcctggcttctgctgcaagagggggatatggagaaggtgggccagggtgtgtggacccgggcagaatctggggaagaagcctgccattcgtctttctttcccacaccaccgaacccactgcccttcccacccccacagcccttttatgaaatcagacaacgtggtaggtggaaaacagcagggcctttcctctgggttttcaaccagaagtgatattccacagttttaactggttactgtgaagtccaagcggccagaattgtgaaaatgtccactgaaacactgcaagcggtgtacttaaagacagtaggccttttagattttgttatatattttttgtagtgctcttcacaagtggaaattttttttttttttttacttttttttaaaagatttttttgtaaagaagggttgtatttagaggccagtagctagagatccaaccagtggacctcttgaagcactaccaggccttaaggccaccatccgagggagactgggaaaactattattcacccaagcctccggaaatgtaatgtaccagcaggcaaaaaacagttcttcatgtagtacaaaatgaaacgaaacaaaaacaaaaacagaaagtaaaaatgaaaccaaaacatttcttaaattctagtgccatagcttttttgtttgtttgttttttgttgttgttttgttttgttcataagaaagagagaaagatactacttatccgtcagacacatgcatcctcatgtggtcgttgaactgctcgatttggtcaaactttgctgggcagacggagcagacgtaagtggtcccctccgtgcaggccaccacgcctggggggccagcgcgggcacctgggggtgtgcctgcagggggggtcccattgctggcactgtgcagggccacgtgtcgctccaggagggtcttgtgagagaacttctttttgcagatgtagcactcgtaggacttctctccccggtggaggcgcatgtgcacgttgagggagctcttctgggtgaagcgcttgttgcagatactacactggtatgccctcactcctgtgtgtgtcaccatgtgcttgataaggtaatcctttaaggagaaggagcgccaacagatgctgcattggtggggcttctcacctgtgtgtacgaacatgtgcttgacgtagttctgtttggcggtgaaagtcttgttgcagagagtgcactcataaggctttttttcgccttgcccactggctgtgctgtggcctgcggatgaggccaggggctgtggcgctggcagctgtgcagtaaaggtcgacagaccgggctgggacactgtcacaaactgggtctgctggcctgccaggggctgtggcaggctgaagaggaaaggcttggggccactgcccgcgggctgggtagtgaagagggctggcaggtaggtgttgccagctgtgccaatgacctgcgtgttgctggtcaaggtcagaggcatcctcaggttgctggtgagggtttctgtctggcgtaagtagagctgggtacttggcaatggctgcccgatggacgtgttgaccgaaggctgttgtaggacgctcttgtcggagctgttgctgacagtgataacagtgctgtccatctccacttcattgcttctctccggagaggaagcacctgtttctagctggtttgtctgcggaccaccctcagcgggggcttctgcagcctgctcgggttgggtgggttcagcctggctgtcccgcgccgccccaggcccaaactgctgctccaccgagtcaggctcggtgcctatggaggagctgacgcccgagtcgaagctttcacctttgggctcactctcggtgccctcggcctggtctgtgtcttccgtgcactcctcggattcgttgcgttccaggatctgcaccctttgctgcccgtagtagtcgtaatcgtcctccatctcctgcttgatgtggatgttgcccactagggtctggatgcgcacaggccggggctgcttgcggcagtgcgtggtctcgggggtggtggacaggtagcgctccatctgctgcgagcgctcatggatgcgtgtgatccagctggggtcttccatgtggtggtcgcggggcaggccgagcgcagtctcgtggtggctgaccactgcgccgctgtaaaaagagcgctcgccgctgccattctgcatggagcacgcgtagagtgccgagtagatcctgtccacgctgtgctgtgggtggctctgcaggtagcccgactccgtgtcgctgctctggcctgacgtgcctgactcgggagtgccccgcggcgtgtcctggcccgagtcctggatccccgggaacacatcgcccacgttctgtgacacgatgcgcgtgcactcgtcgatgactgttttgatctgcaggatgctggcggccgtgaggatctgcagagcttccgactgcgagacccgtagcacgccgctgtacatgaagtcaatgagcttttgcactgactgcactgacaccaccgacgggatctcgatgtcgctgtagccaagcagcagtttgtcctggaagaaggggctgccggctgccagcacgcagcggtgtgcgcgcagcatgctcccgtggatgcgcaccgttacgtcacagaagtggccacggttgcgctgctcgttgagggtctcgagcacggaattgctgaagttgtgaaggttgatgctgtgaatgcgctcggtcatccccttgcaactgatgtcacaatcagatgacccggtgtgagcgtgagagtttgtcagtgaatgtgttgagtggatgagggctgggtctggagacaaaacagcttcaaagttcaggcagggaaggcccggcttggcgctggatccacccggctgagtaatctcattctcctcagatgccttctggttttcagctgtcttgggtttcttcagtagtttcaaaatcaatggtgtcactcttcaggtaaattactccaaggcttgggcctagtgcagatgttcattggggcagggagcagagagcggctgcatgtaaagagaaggggcaggtcacagactgatggtcaaagattctttctgctcgggaggctgaggttcctacatttccagctcatgctggactgtaccgtaagcaacaagt

SEQ ID NO: 16691 - RNA, 13033 nt, Homo sapiens
  source 1..13033: mol_type = other RNA
taaaacccacaattatgtttgtctagtagaaatatatctgctggaacactttggagaacagattggtaattttgccattacactagacattagccctttcaaagcagactaagagtacgtagttccttagtgaatacaaggcttcacaactgaagagcattgcagggagcttggctaaggtgaaaagggacttgctggagaggtacagcagaatgggatgggattagaaaacaacaatctattaggaaagatgaaaggaaggaattccccagtgttcacgctgagaagtcttcatattggaccagtgtgagggggtcttttatactgaggttttaaaaacctgacttcattttgtcctgaatgtagaagtgaagaaggacactagtttcaggcacctgggatggtggaaaagtttattcaactgaggctttccatgcattgggttgaatagctgagggaagctgaagactcttatctgaaaatatgatctgaaaatatttattgtataggaagacagaatgcctgatttctgaagttttcttgatggcccaactaaagaagaaaggcaccaaatcctcactttaacaggtaaatggagatcctgagggctggatacccaagagccaccattttacggattcctcagatttaaaaatgtctcagatagatatttccaaattctatttctattagcctctgtggataaagagttcctgaaactctggttttactttttttggaaaaaaaaaaaaaaaaaaaaaaaaaaaacaactcccaggaaaatgaacactatattgccaagctgcctccagggaaaggttgaagactagttaaaataattctaagcgtattgaaaaaagaaagtgtaaagatccagtattaaaatgaatgtttgagaatacagtggggacaactaggtaattcactgtcttacgcttttcagaagactggccctttgaaacgcagcctgttattgttggtcagatcatgtggcacttaagtagccccttggtcatatttttaaaagcaaatatagacagtgacagtcctacaggggaaaatcacagatacattcatatgcacctcttttgttcttcagatattgagtgggtcagctaaacaagatcactttgaatatgaacctctttgtattagtcacaccaacaaaaaagtttcaaaaaaagttttcactttcctacatttgctaagtctgagctttaaaaaattctaaaatcctctaaagacaatactgaagctgataatataaaaagcaaattagagcactaatgattattactagatgcaccagattaactgcagcaggttggtgatgggtgatataagcaaagacataatatttcaatcaactcatgatcataggcagattcaaaagttaaaatgaatataatgtaatatatatttcaatatagagttgttatatataatgtgtatgtcctaggtttcagaaatactgcaatgtagtgtattgtagttaagtaagcatacctaaatagtaactcatattctttcacaaagtcactagtactgttaattaaaggaaaaaataaaaccgaaacaactaattgtttttccagtaaaaagaaatacctatggttacagttacagacttcttttggatatagaaagacaatatacattttaaaaagtaataacgacaaaaaagttgcaactgtaagtagccttacttaacaggggaaggggaaaagtcaccagaatagaagaggaaagaaaatgtcctctgacttctgtaaaacagaaataatgtacaaatcataaaaaataacaaaccatctagtaaaagaagggcatgggagtgagaaaactgaatcctgaattccaggccaccaaaccctcagagtccattcattcagtatattatactagagtggcattctacttcaatgcttgagatgggcaagagcaatcaattcctacagattaccaaaaaacattccccccaacagtctattggtttgctagacatggtaaacaacccactcctggaaagactttggcaaaggccacattggtttcaggagacacagtttgtgaattacgatgatatcttgtgagtacaggcagaattaggaagctttagtttgagaataaaatttatgtgtgtgtgtgtgtgtgtgtgtgtgtgtgtgcacactgcattgcatagaggaaaggaatgaagacctttgagctatgggatggctcaggccaaagtttgtgtgggctttgcctgcctggcattggtccccacccctgccacctccaggagacctggggagacgccctggactgctgctccctcttgtctgctcaccagttgaagacttctgttataccttattatggaggaaaacagcctgtccctgtgggtttgctgtggattcaacaagctgcatttgtttctcccaattctgaaacattacaaaaagcaacagagtgggcaggtgactgcttcctgggaagggagccacaagtcttaaacacaatggtgggaagaggcaactgtatctatgcacgaggacctctgcctgtgtgtgcttcctttggggggcacacacacttccagatgacaataagtatatacacaaacacacacatgtgcacacatgtcaataaatccaatagaactgtagagtttgttaaatgcactctactccacataagcatattcaagtttctcatgaaacggatacatagaaattactgatggttgggctccttcagaatgccctaaagtctcatcacagatactgatgcacccaactaaggcaacaaagcataagcagatacgtgagatatgtcagaccttcgacttctaaccagaagttcaaaaatgtatcttgttgtcactgggcaatatgaatgtgaaacagttttgtgctgagggaagctcacactgtgtgtgcacatgtataaataatgtatactcatttatagacattttggacagcagcggtgacatactggatgggttaagactctttcattattagaatctacatataaattgcaatgagtttgctgggtaaaaacaactgttgcaacactagtagaaacagatgcccccaaggtttttttttttttttttttttttttctctcttggatgtatcaaaatctcattgaggcattctaaaccaaagaaacctctgaatttgaaacagggttagtagggacttttatacccagctgggcatcccagaagcctggactctcaggactgtggctagattttgcccatgatctgtagattatgctcttgcaccggagacttgaaagttatgagtttgcattcaaacaaagaaccaccagataaaacagatgttctctaaaactgaggaaaaaaagtttagagatatacactgtatagagaaagaaagctttttgctggattgttctccttgttaaggaaatgtttaaaactagtactcccgggcacctgtgattgcattttataggattctatttagtaatatgatgtctattttacattcagccccaacctacgtcactgaaatagaataggaaatagcagccactatctgagagtacccagttctaggaaagtttggtgcctcctcaagaagtcactatttccatagtcctcaatcatgaatagggcttgtttttgtgataatgtaactattaaacagcaagaaatgcctataacttcagagccttctcatttctatatcttttatcctcttcccagggctttctgatttaaggcaataatgctacactataagtagccttttgtgaaaataccttaattgaggtcacttaagattagatttcagtctgaaagtctacagtttacggagcaaaaggtggagcctaaagaaaccactggcaggtgttttagtcagtggtgtggaaagataatgtttcttgtttcaacccagggcatttttacccatcatgcagtgaggagaaaatacatagttctgaaaaagaacccacactaggtagccctaattttctatctcttcactctaaaaaggatggaaacaagccctactgttccataaccattcccagggatcggctaaggtacattgctgactgctatagactcagtgttcaaggagaaaaaaatcttcagagacttagaaaactctttgcaatattttggtcaggctgatcgtcttgatactcagtgctagaaatgatgctttggattagtagtttccacattctgaatttataggaacactgagtcaccacagccttttttcttgtaaaggtttaagtgatatcagaaatagcaactctacacggaaagcccttgggaatatgaaaatactctctctcaagagcaagggctcttccgtgccccttttctgcctctgtatgtagcctgagcaccagggtagagattgcttttgaaagtttgccccatgtaatctatttcctggctacctaagagaacagccgttttcttcatgaaaacacaaagaggggaaagaggctgctgctgttccagtgggaagttatgtctagccccagaaggcctggtggctgggtcagctcaagcactctcttcatgcactgcaggctcaggaggcattgggttgctttgctttttctatggaattagggagcctattgaaattctagtgcacccctccttttgtttgtcaccaagtcacatggttctgtcttcagtatcctatttttctttttttttaatttctttttctgaggaacaaaattggccatttaaataaagttcttttctagtgagtaaagaggtttctcagagccagaaatcactgaaaagagagtctgtcgaccctgcccatggaaaagcccagagatttctctaaccacttcttgccaaacttcctagttttgtgattggatgtttcttggtttagcattgtttggtgctgaatacattttgcaattcttttgttctctgccctagagcttccattaccctggacttcaactcattaccaaattaaagaattcttttagaagatttcttttaagagtcaggtcacaacagaaagggcgccctcctgttctcctaaatctcaagggcatctcaggttgtgtctgctcttacgttgcaccttccttttgttcccttttaatgcagcagcacactggctatagcagaggcagacctgatttgattatctgataccttttccacaaaatcatatatcccctgctcccagccccaactaatcaaataacatcttctagaacaacagaggaaagctccagaatgggtgtatatcctgtgactcctggccagatccaccttgctccctgtcttcctaggggtcacaggtgttgggagcattgtggaggagccccaacaaggaagcaacatatggctttattatgttttctcaggaatcgaaggggttttataaggggcatatctcatttttgacttctgtgctgagagaaaatattgagttttgggcgcaggcagagcacagacaggacagctggtgttcctgtgtgagggaagtacacatagctcaaggctttaggactgaatgtgaaacaaacatacctggaggaaaacttttttcattatcagaattcacaaattcttactgttcatgggttgaaaaagagtatttgggaccttatagaatattttgatgatacaaaataaaacccttatgacttttaaacacagcaaacccaagtctttctaaggccaagagctactatgatctctaagatgactaggaatgaactgaggctagaatatgagcaggaaattatccagcacacttaatcatggcacaaatagattcaaagcattaggaatttgggaagagaacggtctataaaactgttattaggagctaaagtttacctctcaattaaaagatacaggaaaccattttgatacagagattttcatttcagattttttttctttgcttagcttgtttccccctgtgtagaattgtaacagatccatgtgttccaattattttcttttttaggattatatttcacacatttgggggccttttttgtacaaatattggcatgtaataaggaaaaattgcccatgatgctgagataataccagtgtttttagtggtagaaaatattatttttttataaaccatatctaaatatcttgagataaaaattcccctttgactttttttcctctcccttgtttggcaaattccattttaaaattataaattgctaaaaaatgtcctttccatactatttctctcttccttgtactcatcctaagaagtcttaaatctggaacatttgcttttatcttatctatctgtttcctggctactagaaagaaatttttttagcactcatatcaccctaccatgaaggtctaaatgtaagatgactgtaggacttgaaacaaaaaaaaattaaaaagatccacactcattctttgattttgaagcaaatgtctttccctatttctaaagatatttgtgattgtttaacttaaaagtgagaattgacaatctaaaagcatctctatccttttgaaacaggtccagattggtttatttcctaaaatgtgggtcagtttggaaagtggccatttgatgggccaggaacatagcaataaacaactacctctttgctcctccagattagatctcccactccaatccagcttcttcctctttccacaaaataatttgtcaactattttagaatgtgacatatttgggaaggataaatgtacagtaggaatatgtctactgctatgcaaacctggctggtccattttgtcatggactacaatgattatatcacctcattaagaattctttagggatcctccacctcctcccccactcccttttttttaagagacacttcctttacagggaaaggatgatagactcctcagggtttcaagtcacctgcagctttttctctacatgttctaccaaaagaaaaggtggattctaacccaattgcttagcattttacatggcaaatcagcattaaggcaaatgggtctctctcagatttgagaaacagaaagctacacgtggcccataatggcacctaagatcaacttttcaggcggtattagtgaaaattcttcctactttgctaaatttgaacaaagacactttcaaatctactgtgaaacagtttaaaatattttaaagtggcttttggccttctttcatttgtaacatgtattgagtgatttcatgtcattgtctcctagctttaagagtttttttcttaaggtcaatcttctcttttcattttatgggtggaatcacttgttttccaaaatatcaaaacaattccatgacatagttaattaatgctccctctattggtggtaagtggaaatattagtcttacaacactgctattttaaaaagcaaaattagcaatagaaaaatgaacttactttatctcggaagctgttcctcactaactgttaaaacagatcagttttggacatacagttcttggcaggactcctcttagaaatcacaataggttacacttaatagtcagttaaccacccaagtttacattaaaacttctagcaaaatatccactgaattaagcactgtgggaccaaatcaaactcacaaacacttcagttacactaaccttacaaagcatcacaaagaacttatgaaaaagatccaagttaaccaaatgtctaaaatatatgaataaaaccaatttagtcattacagagttgtttgtgttggaagattttccctcgtttgctgcacagtttttgtaaataaaatgctgacaggaaaattagaaggaaaattaaattaaaatgtaatgtaattttgaaactaaaatacgctctcctttcttctttttaaaactgtagtttggtgttttgctttgtttaaagatttgctttcccctaagtatgttaaaatatgcccagcaatgaaatcactttgggagtttcagctaggtttaagaattcctatatttgagctggaatcccttcaggacactgtctataatgaaaatgtctctattataacaccttgatcaggaccgaggagagaaatccctactaggaagagagagtggcatctggtatgatgcaatagattggtggtcttttgaatggtggctgttggcatctgggaatttttttgttaatttccctaaaacctttcgaagaagcaagggttaattcgtcatctaaagaatgatcatcttattcagccctcttaaccatggtggaaacagtcagaaggtgatatttggaaggaaaaaagtaattttggcatcaatgcatcttgatctataacaggcttctcataatgatgctctttgtagttgggaagggtgaggagctatggcagagttttgtgaactcctcttcctggctgatcacaaaagaaaagaccccatttatcaagacttctagactattagtgtttcactaagaaaaaaagtaaagtcaatagaaattctagaattgtaagatctcaatgaaattttggagaagcaagcaatctctttctgaaagataaagtctcttccatgaaaaagaacagaattctagatgaatcagttgaaaaaattattcagtggggcaacttaagcttgctaaagtcaaagaactacatatcaaaatacaaagcagcaattcaaattacagcagggatgggctggccacagaggccctcatcaacccaggcaatacttaaaataataaaaattaagaaaaattaaaaaaaatatgaagaaaatatccttcctctctttcaaatataactttagttgccttttattctttctatctggaagcagtatcgctaaccttaacagtcttgacttaccaaaaaatatatatatgtgtgtgaaataaaataaaagagaaggaattggtggcagtgtatgcaaaaccaaaatgaaaaaaattacttttaacaatttcactttttttgtttttttttttacacaaatactgttgtaaatatattaaaaaaatcagcattctatctggtaaacgtcacttttgcccctctataaaattttgaattaaaaaagcctcaagaactttttattgttccccccaccctccatttctttttctttttctcttccacaagaatatatcctgacactttttttttttttgcaaagattgttggaaataatccttctcttgtacctagaaacataggtgcaaatttctgatatctttgttttatctgcattcctgcctttcatgaaagtccctcttgattgtgctgaggctgtggctcagcgaagacactgaataaatacgatagccactgttgcttgttgcttgtccaagtcttcctggcttctgctgcaagagggggatatggagaaggtgggccagggtgtgtggacccgggcagaatctggggaagaagcctgccattcgtctttctttcccacaccaccgaacccactgcccttcccacccccacagcccttttatgaaatcagacaacgtggtaggtggaaaacagcagggcctttcctctgggttttcaaccagaagtgatattccacagttttaactggttactgtgaagtccaagcggccagaattgtgaaaatgtccactgaaacactgcaagcggtgtacttaaagacagtaggccttttagattttgttatatattttttgtagtgctcttcacaagtggaaattttttttttttttttacttttttttaaaagatttttttgtaaagaagggttgtatttagaggccagtagctagagatccaaccagtggacctcttgaagcactaccaggccttaaggccaccatccgagggagactgggaaaactattattcacccaagcctccggaaatgtaatgtaccagcaggcaaaaaacagttcttcatgtagtacaaaatgaaacgaaacaaaaacaaaaacagaaagtaaaaatgaaaccaaaacatttcttaaattctagtgccatagcttttttgtttgtttgttttttgttgttgttttgttttgttcataagaaagagagaaagatactacttatccgtcagacacatgcatcctcatgtggtcgttgaactgctcgatttggtcaaactttgctgggcagacggagcagacgtaagtggtcccctccgtgcaggccaccacgcctggggggccagcgcgggcacctgggggtgtgcctgcagggggggtcccattgctggcactgtgcagggccacgtgtcgctccaggagggtcttgtgagagaacttctttttgcagatgtagcactcgtaggacttctctccccggtggaggcgcatgtgcacgttgagggagctcttctgggtgaagcgcttgttgcagatactacactggtatgccctcactcctgtgtgtgtcaccatgtgcttgataaggtaatcctttaaggagaaggagcgccaacagatgctgcattggtggggcttctcacctgtgtgtacgaacatgtgcttgacgtagttctgtttggcggtgaaagtcttgttgcagagagtgcactcataaggctttttttcgccttgcccactggctgtgctgtggcctgcggatgaggccaggggctgtggcgctggcagctgtgcagtaaaggtcgacagaccgggctgggacactgtcacaaactgggtctgctggcctgccaggggctgtggcaggctgaagaggaaaggcttggggccactgcccgcgggctgggtagtgaagagggctggcaggtaggtgttgccagctgtgccaatgacctgcgtgttgctggtcaaggtcagaggcatcctcaggttgctggtgagggtttctgtctggcgtaagtagagctgggtacttggcaatggctgcccgatggacgtgttgaccgaaggctgttgtaggacgctcttgtcggagctgttgctgacagtgataacagtgctgtccatctccacttcattgcttctctccggagaggaagcacctgtttctagctggtttgtctgcggaccaccctcagcgggggcttctgcagcctgctcgggttgggtgggttcagcctggctgtcccgcgccgccccaggcccaaactgctgctccaccgagtcaggctcggtgcctatggaggagctgacgcccgagtcgaagctttcacctttgggctcactctcggtgccctcggcctggtctgtgtcttccgtgcactcctcggattcgttgcgttccaggatctgcaccctttgctgcccgtagtagtcgtaatcgtcctccatctcctgcttgatgtggatgttgcccactagggtctggatgcgcacaggccggggctgcttgcggcagtgcgtggtctcgggggtggtggacaggtagcgctccatctgctgcgagcgctcatggatgcgtgtgatccagctggggtcttccatgtggtggtcgcggggcaggccgagcgcagtctcgtggtggctgaccactgcgccgctgtaaaaagagcgctcgccgctgccattctgcatggagcacgcgtagagtgccgagtagatcctgtccacgctgtgctgtgggtggctctgcaggtagcccgactccgtgtcgctgctctggcctgacgtgcctgactcgggagtgccccgcggcgtgtcctggcccgagtcctggatccccgggaacacatcgcccacgttctgtgacacgatgcgcgtgcactcgtcgatgactgttttgatctgcaggatgctggcggccgtgaggatctgcagagcttccgactgcgagacccgtagcacgccgctgtacatgaagtcaatgagcttttgcactgactgcactgacaccaccgacgggatctcgatgtcgctgtagccaagcagcagtttgtcctggaagaaggggctgccggctgccagcacgcagcggtgtgcgcgcagcatgctcccgtggatgcgcaccgttacgtcacagaagtggccacggttgcgctgctcgttgagggtctcgagcacggaattgctgaagttgtgaaggttgatgctgtgaatgcgctcggtcatccccttgcaactgatgtcacaatcagatgacccggtgtgagcgtgagagtttgtcagtgaatgtgttgagtggatgagggctgggtctggagacaaaacagcttcaaagttcaggcagggaaggcccggcttggcgctggatccacccggctgagtaatctcattctcctcagatgccttctggttttcagctgtcttgggtttcttccgttctagcatttgtcaggaagcttagagacaggactcgtggagtaatgggaggagcactggactgggagtcaggagacttgagctaccgtactagctgtgcctctaacttgctgtgtggccttgggcacctcacttcacctctctgggcttcagtttcctcatagtagtttcaaaatcaatggtgtcactcttcaggtaaattactccaaggcttgggcctagtgcagatgttcattggggcagggagcagagagcggctgcatgtaaagagaaggggcaggtcacagactgatggtcaaagatcagacagcaatgtcatgaggaatatcctgttagtaatgatgaaacattaggaatacagtgcagctcaatcttttgtttttaaggtgcagtgatttcagtctctaaatgtaacttcaggcagtctgtgcagctatggggcacaaacttgcaattcatcaattcttcagccttcagagtcccaaaggcaattcttaacacttctttttatttgtagtggcatggatgacggagcagaaatagagaattcttgattaaccaggagaagaatatcataggcatgggtgtgagatcaactggagattcaaggaagctaaagtgcccagaatgaactaatgttgtaatgtagactgtgagcagagataaaattccagaagccaaggagtgttgtacggtaagtcctggcagtgcctcctcgcgctctttaatcttctttcctcaactcctaaacttccccccgcccctacttcttcggcagaag

SEQ ID NO: 16692 - RNA, 12441 nt, Homo sapiens
  source 1..12441: mol_type = other RNA
taaaacccacaattatgtttgtctagtagaaatatatctgctggaacactttggagaacagattggtaattttgccattacactagacattagccctttcaaagcagactaagagtacgtagttccttagtgaatacaaggcttcacaactgaagagcattgcagggagcttggctaaggtgaaaagggacttgctggagaggtacagcagaatgggatgggattagaaaacaacaatctattaggaaagatgaaaggaaggaattccccagtgttcacgctgagaagtcttcatattggaccagtgtgagggggtcttttatactgaggttttaaaaacctgacttcattttgtcctgaatgtagaagtgaagaaggacactagtttcaggcacctgggatggtggaaaagtttattcaactgaggctttccatgcattgggttgaatagctgagggaagctgaagactcttatctgaaaatatgatctgaaaatatttattgtataggaagacagaatgcctgatttctgaagttttcttgatggcccaactaaagaagaaaggcaccaaatcctcactttaacaggtaaatggagatcctgagggctggatacccaagagccaccattttacggattcctcagatttaaaaatgtctcagatagatatttccaaattctatttctattagcctctgtggataaagagttcctgaaactctggttttactttttttggaaaaaaaaaaaaaaaaaaaaaaaaaaaacaactcccaggaaaatgaacactatattgccaagctgcctccagggaaaggttgaagactagttaaaataattctaagcgtattgaaaaaagaaagtgtaaagatccagtattaaaatgaatgtttgagaatacagtggggacaactaggtaattcactgtcttacgcttttcagaagactggccctttgaaacgcagcctgttattgttggtcagatcatgtggcacttaagtagccccttggtcatatttttaaaagcaaatatagacagtgacagtcctacaggggaaaatcacagatacattcatatgcacctcttttgttcttcagatattgagtgggtcagctaaacaagatcactttgaatatgaacctctttgtattagtcacaccaacaaaaaagtttcaaaaaaagttttcactttcctacatttgctaagtctgagctttaaaaaattctaaaatcctctaaagacaatactgaagctgataatataaaaagcaaattagagcactaatgattattactagatgcaccagattaactgcagcaggttggtgatgggtgatataagcaaagacataatatttcaatcaactcatgatcataggcagattcaaaagttaaaatgaatataatgtaatatatatttcaatatagagttgttatatataatgtgtatgtcctaggtttcagaaatactgcaatgtagtgtattgtagttaagtaagcatacctaaatagtaactcatattctttcacaaagtcactagtactgttaattaaaggaaaaaataaaaccgaaacaactaattgtttttccagtaaaaagaaatacctatggttacagttacagacttcttttggatatagaaagacaatatacattttaaaaagtaataacgacaaaaaagttgcaactgtaagtagccttacttaacaggggaaggggaaaagtcaccagaatagaagaggaaagaaaatgtcctctgacttctgtaaaacagaaataatgtacaaatcataaaaaataacaaaccatctagtaaaagaagggcatgggagtgagaaaactgaatcctgaattccaggccaccaaaccctcagagtccattcattcagtatattatactagagtggcattctacttcaatgcttgagatgggcaagagcaatcaattcctacagattaccaaaaaacattccccccaacagtctattggtttgctagacatggtaaacaacccactcctggaaagactttggcaaaggccacattggtttcaggagacacagtttgtgaattacgatgatatcttgtgagtacaggcagaattaggaagctttagtttgagaataaaatttatgtgtgtgtgtgtgtgtgtgtgtgtgtgtgtgcacactgcattgcatagaggaaaggaatgaagacctttgagctatgggatggctcaggccaaagtttgtgtgggctttgcctgcctggcattggtccccacccctgccacctccaggagacctggggagacgccctggactgctgctccctcttgtctgctcaccagttgaagacttctgttataccttattatggaggaaaacagcctgtccctgtgggtttgctgtggattcaacaagctgcatttgtttctcccaattctgaaacattacaaaaagcaacagagtgggcaggtgactgcttcctgggaagggagccacaagtcttaaacacaatggtgggaagaggcaactgtatctatgcacgaggacctctgcctgtgtgtgcttcctttggggggcacacacacttccagatgacaataagtatatacacaaacacacacatgtgcacacatgtcaataaatccaatagaactgtagagtttgttaaatgcactctactccacataagcatattcaagtttctcatgaaacggatacatagaaattactgatggttgggctccttcagaatgccctaaagtctcatcacagatactgatgcacccaactaaggcaacaaagcataagcagatacgtgagatatgtcagaccttcgacttctaaccagaagttcaaaaatgtatcttgttgtcactgggcaatatgaatgtgaaacagttttgtgctgagggaagctcacactgtgtgtgcacatgtataaataatgtatactcatttatagacattttggacagcagcggtgacatactggatgggttaagactctttcattattagaatctacatataaattgcaatgagtttgctgggtaaaaacaactgttgcaacactagtagaaacagatgcccccaaggtttttttttttttttttttttttttctctcttggatgtatcaaaatctcattgaggcattctaaaccaaagaaacctctgaatttgaaacagggttagtagggacttttatacccagctgggcatcccagaagcctggactctcaggactgtggctagattttgcccatgatctgtagattatgctcttgcaccggagacttgaaagttatgagtttgcattcaaacaaagaaccaccagataaaacagatgttctctaaaactgaggaaaaaaagtttagagatatacactgtatagagaaagaaagctttttgctggattgttctccttgttaaggaaatgtttaaaactagtactcccgggcacctgtgattgcattttataggattctatttagtaatatgatgtctattttacattcagccccaacctacgtcactgaaatagaataggaaatagcagccactatctgagagtacccagttctaggaaagtttggtgcctcctcaagaagtcactatttccatagtcctcaatcatgaatagggcttgtttttgtgataatgtaactattaaacagcaagaaatgcctataacttcagagccttctcatttctatatcttttatcctcttcccagggctttctgatttaaggcaataatgctacactataagtagccttttgtgaaaataccttaattgaggtcacttaagattagatttcagtctgaaagtctacagtttacggagcaaaaggtggagcctaaagaaaccactggcaggtgttttagtcagtggtgtggaaagataatgtttcttgtttcaacccagggcatttttacccatcatgcagtgaggagaaaatacatagttctgaaaaagaacccacactaggtagccctaattttctatctcttcactctaaaaaggatggaaacaagccctactgttccataaccattcccagggatcggctaaggtacattgctgactgctatagactcagtgttcaaggagaaaaaaatcttcagagacttagaaaactctttgcaatattttggtcaggctgatcgtcttgatactcagtgctagaaatgatgctttggattagtagtttccacattctgaatttataggaacactgagtcaccacagccttttttcttgtaaaggtttaagtgatatcagaaatagcaactctacacggaaagcccttgggaatatgaaaatactctctctcaagagcaagggctcttccgtgccccttttctgcctctgtatgtagcctgagcaccagggtagagattgcttttgaaagtttgccccatgtaatctatttcctggctacctaagagaacagccgttttcttcatgaaaacacaaagaggggaaagaggctgctgctgttccagtgggaagttatgtctagccccagaaggcctggtggctgggtcagctcaagcactctcttcatgcactgcaggctcaggaggcattgggttgctttgctttttctatggaattagggagcctattgaaattctagtgcacccctccttttgtttgtcaccaagtcacatggttctgtcttcagtatcctatttttctttttttttaatttctttttctgaggaacaaaattggccatttaaataaagttcttttctagtgagtaaagaggtttctcagagccagaaatcactgaaaagagagtctgtcgaccctgcccatggaaaagcccagagatttctctaaccacttcttgccaaacttcctagttttgtgattggatgtttcttggtttagcattgtttggtgctgaatacattttgcaattcttttgttctctgccctagagcttccattaccctggacttcaactcattaccaaattaaagaattcttttagaagatttcttttaagagtcaggtcacaacagaaagggcgccctcctgttctcctaaatctcaagggcatctcaggttgtgtctgctcttacgttgcaccttccttttgttcccttttaatgcagcagcacactggctatagcagaggcagacctgatttgattatctgataccttttccacaaaatcatatatcccctgctcccagccccaactaatcaaataacatcttctagaacaacagaggaaagctccagaatgggtgtatatcctgtgactcctggccagatccaccttgctccctgtcttcctaggggtcacaggtgttgggagcattgtggaggagccccaacaaggaagcaacatatggctttattatgttttctcaggaatcgaaggggttttataaggggcatatctcatttttgacttctgtgctgagagaaaatattgagttttgggcgcaggcagagcacagacaggacagctggtgttcctgtgtgagggaagtacacatagctcaaggctttaggactgaatgtgaaacaaacatacctggaggaaaacttttttcattatcagaattcacaaattcttactgttcatgggttgaaaaagagtatttgggaccttatagaatattttgatgatacaaaataaaacccttatgacttttaaacacagcaaacccaagtctttctaaggccaagagctactatgatctctaagatgactaggaatgaactgaggctagaatatgagcaggaaattatccagcacacttaatcatggcacaaatagattcaaagcattaggaatttgggaagagaacggtctataaaactgttattaggagctaaagtttacctctcaattaaaagatacaggaaaccattttgatacagagattttcatttcagattttttttctttgcttagcttgtttccccctgtgtagaattgtaacagatccatgtgttccaattattttcttttttaggattatatttcacacatttgggggccttttttgtacaaatattggcatgtaataaggaaaaattgcccatgatgctgagataataccagtgtttttagtggtagaaaatattatttttttataaaccatatctaaatatcttgagataaaaattcccctttgactttttttcctctcccttgtttggcaaattccattttaaaattataaattgctaaaaaatgtcctttccatactatttctctcttccttgtactcatcctaagaagtcttaaatctggaacatttgcttttatcttatctatctgtttcctggctactagaaagaaatttttttagcactcatatcaccctaccatgaaggtctaaatgtaagatgactgtaggacttgaaacaaaaaaaaattaaaaagatccacactcattctttgattttgaagcaaatgtctttccctatttctaaagatatttgtgattgtttaacttaaaagtgagaattgacaatctaaaagcatctctatccttttgaaacaggtccagattggtttatttcctaaaatgtgggtcagtttggaaagtggccatttgatgggccaggaacatagcaataaacaactacctctttgctcctccagattagatctcccactccaatccagcttcttcctctttccacaaaataatttgtcaactattttagaatgtgacatatttgggaaggataaatgtacagtaggaatatgtctactgctatgcaaacctggctggtccattttgtcatggactacaatgattatatcacctcattaagaattctttagggatcctccacctcctcccccactcccttttttttaagagacacttcctttacagggaaaggatgatagactcctcagggtttcaagtcacctgcagctttttctctacatgttctaccaaaagaaaaggtggattctaacccaattgcttagcattttacatggcaaatcagcattaaggcaaatgggtctctctcagatttgagaaacagaaagctacacgtggcccataatggcacctaagatcaacttttcaggcggtattagtgaaaattcttcctactttgctaaatttgaacaaagacactttcaaatctactgtgaaacagtttaaaatattttaaagtggcttttggccttctttcatttgtaacatgtattgagtgatttcatgtcattgtctcctagctttaagagtttttttcttaaggtcaatcttctcttttcattttatgggtggaatcacttgttttccaaaatatcaaaacaattccatgacatagttaattaatgctccctctattggtggtaagtggaaatattagtcttacaacactgctattttaaaaagcaaaattagcaatagaaaaatgaacttactttatctcggaagctgttcctcactaactgttaaaacagatcagttttggacatacagttcttggcaggactcctcttagaaatcacaataggttacacttaatagtcagttaaccacccaagtttacattaaaacttctagcaaaatatccactgaattaagcactgtgggaccaaatcaaactcacaaacacttcagttacactaaccttacaaagcatcacaaagaacttatgaaaaagatccaagttaaccaaatgtctaaaatatatgaataaaaccaatttagtcattacagagttgtttgtgttggaagattttccctcgtttgctgcacagtttttgtaaataaaatgctgacaggaaaattagaaggaaaattaaattaaaatgtaatgtaattttgaaactaaaatacgctctcctttcttctttttaaaactgtagtttggtgttttgctttgtttaaagatttgctttcccctaagtatgttaaaatatgcccagcaatgaaatcactttgggagtttcagctaggtttaagaattcctatatttgagctggaatcccttcaggacactgtctataatgaaaatgtctctattataacaccttgatcaggaccgaggagagaaatccctactaggaagagagagtggcatctggtatgatgcaatagattggtggtcttttgaatggtggctgttggcatctgggaatttttttgttaatttccctaaaacctttcgaagaagcaagggttaattcgtcatctaaagaatgatcatcttattcagccctcttaaccatggtggaaacagtcagaaggtgatatttggaaggaaaaaagtaattttggcatcaatgcatcttgatctataacaggcttctcataatgatgctctttgtagttgggaagggtgaggagctatggcagagttttgtgaactcctcttcctggctgatcacaaaagaaaagaccccatttatcaagacttctagactattagtgtttcactaagaaaaaaagtaaagtcaatagaaattctagaattgtaagatctcaatgaaattttggagaagcaagcaatctctttctgaaagataaagtctcttccatgaaaaagaacagaattctagatgaatcagttgaaaaaattattcagtggggcaacttaagcttgctaaagtcaaagaactacatatcaaaatacaaagcagcaattcaaattacagcagggatgggctggccacagaggccctcatcaacccaggcaatacttaaaataataaaaattaagaaaaattaaaaaaaatatgaagaaaatatccttcctctctttcaaatataactttagttgccttttattctttctatctggaagcagtatcgctaaccttaacagtcttgacttaccaaaaaatatatatatgtgtgtgaaataaaataaaagagaaggaattggtggcagtgtatgcaaaaccaaaatgaaaaaaattacttttaacaatttcactttttttgtttttttttttacacaaatactgttgtaaatatattaaaaaaatcagcattctatctggtaaacgtcacttttgcccctctataaaattttgaattaaaaaagcctcaagaactttttattgttccccccaccctccatttctttttctttttctcttccacaagaatatatcctgacactttttttttttttgcaaagattgttggaaataatccttctcttgtacctagaaacataggtgcaaatttctgatatctttgttttatctgcattcctgcctttcatgaaagtccctcttgattgtgctgaggctgtggctcagcgaagacactgaataaatacgatagccactgttgcttgttgcttgtccaagtcttcctggcttctgctgcaagagggggatatggagaaggtgggccagggtgtgtggacccgggcagaatctggggaagaagcctgccattcgtctttctttcccacaccaccgaacccactgcccttcccacccccacagcccttttatgaaatcagacaacgtggtaggtggaaaacagcagggcctttcctctgggttttcaaccagaagtgatattccacagttttaactggttactgtgaagtccaagcggccagaattgtgaaaatgtccactgaaacactgcaagcggtgtacttaaagacagtaggccttttagattttgttatatattttttgtagtgctcttcacaagtggaaattttttttttttttttacttttttttaaaagatttttttgtaaagaagggttgtatttagaggccagtagctagagatccaaccagtggacctcttgaagcactaccaggccttaaggccaccatccgagggagactgggaaaactattattcacccaagcctccggaaatgtaatgtaccagcaggcaaaaaacagttcttcatgtagtacaaaatgaaacgaaacaaaaacaaaaacagaaagtaaaaatgaaaccaaaacatttcttaaattctagtgccatagcttttttgtttgtttgttttttgttgttgttttgttttgttcataagaaagagagaaagatactacttatccgtcagacacatgcatcctcatgtggtcgttgaactgctcgatttggtcaaactttgctgggcagacggagcagacgtaagtggtcccctccgtgcaggccaccacgcctggggggccagcgcgggcacctgggggtgtgcctgcagggggggtcccattgctggcactgtgcagggccacgtgtcgctccaggagggtcttgtgagagaacttctttttgcagatgtagcactcgtaggacttctctccccggtggaggcgcatgtgcacgttgagggagctcttctgggtgaagcgcttgttgcagatactacactggtatgccctcactcctgtgtgtgtcaccatgtgcttgataaggtaatcctttaaggagaaggagcgccaacagatgctgcattggtggggcttctcacctgtgtgtacgaacatgtgcttgacgtagttctgtttggcggtgaaagtcttgttgcagagagtgcactcataaggctttttttcgccttgcccactggctgtgctgtggcctgcggatgaggccaggggctgtggcgctggcagctgtgcagtaaaggtcgacagaccgggctgggacactgtcacaaactgggtctgctggcctgccaggggctgtggcaggctgaagaggaaaggcttggggccactgcccgcgggctgggtagtgaagagggctggcaggtaggtgttgccagctgtgccaatgacctgcgtgttgctggtcaaggtcagaggcatcctcaggttgctggtgagggtttctgtctggcgtaagtagagctgggtacttggcaatggctgcccgatggacgtgttgaccgaaggctgttgtaggacgctcttgtcggagctgttgctgacagtgataacagtgctgtccatctccacttcattgcttctctccggagaggaagcacctgtttctagctggtttgtctgcggaccaccctcagcgggggcttctgcagcctgctcgggttgggtgggttcagcctggctgtcccgcgccgccccaggcccaaactgctgctccaccgagtcaggctcggtgcctatggaggagctgacgcccgagtcgaagctttcacctttgggctcactctcggtgccctcggcctggtctgtgtcttccgtgcactcctcggattcgttgcgttccaggatctgcaccctttgctgcccgtagtagtcgtaatcgtcctccatctcctgcttgatgtggatgttgcccactagggtctggatgcgcacaggccggggctgcttgcggcagtgcgtggtctcgggggtggtggacaggtagcgctccatctgctgcgagcgctcatggatgcgtgtgatccagctggggtcttccatgtggtggtcgcggggcaggccgagcgcagtctcgtggtggctgaccactgcgccgctgtaaaaagagcgctcgccgctgccattctgcatggagcacgcgtagagtgccgagtagatcctgtccacgctgtgctgtgggtggctctgcaggtagcccgactccgtgtcgctgctctggcctgacgtgcctgactcgggagtgccccgcggcgtgtcctggcccgagtcctggatccccgggaacacatcgcccacgttctgtgacacgatgcgcgtgcactcgtcgatgactgttttgatctgcaggatgctggcggccgtgaggatctgcagagcttccgactgcgagacccgtagcacgccgctgtacatgaagtcaatgagcttttgcactgactgcactgacaccaccgacgggatctcgatgtcgctgtagccaagcagcagtttgtcctggaagaaggggctgccggctgccagcacgcagcggtgtgcgcgcagcatgctcccgtggatgcgcaccgttacgtcacagaagtggccacggttgcgctgctcgttgagggtctcgagcacggaattgctgaagttgtgaaggttgatgctgtgaatgcgctcggtcatccccttgcaactgatgtcacaatcagatgacccggtgtgagcgtgagagtttgtcagtgaatgtgttgagtggatgagggctgggtctggagacaaaacagcttcaaagttcaggcagggaaggcccggcttggcgctggatccacccggctgagtaatctcattctcctcagatgccttctggttttcagctgtcttgggtttcttccgttctagcatttgtcaggaagcttagagacaggactcgtggagtaatgggaggagcactggactgggagtcaggagacttgagctaccgtactagctgtgcctctaacttgctgtgtggccttgggcacctcacttcacctctctgggcttcagtttcctcatccttataccactgggctgtttcccaac

SEQ ID NO: 16693 - RNA, 13156 nt, Homo sapiens
  source 1..13156: mol_type = other RNA
taaaacccacaattatgtttgtctagtagaaatatatctgctggaacactttggagaacagattggtaattttgccattacactagacattagccctttcaaagcagactaagagtacgtagttccttagtgaatacaaggcttcacaactgaagagcattgcagggagcttggctaaggtgaaaagggacttgctggagaggtacagcagaatgggatgggattagaaaacaacaatctattaggaaagatgaaaggaaggaattccccagtgttcacgctgagaagtcttcatattggaccagtgtgagggggtcttttatactgaggttttaaaaacctgacttcattttgtcctgaatgtagaagtgaagaaggacactagtttcaggcacctgggatggtggaaaagtttattcaactgaggctttccatgcattgggttgaatagctgagggaagctgaagactcttatctgaaaatatgatctgaaaatatttattgtataggaagacagaatgcctgatttctgaagttttcttgatggcccaactaaagaagaaaggcaccaaatcctcactttaacaggtaaatggagatcctgagggctggatacccaagagccaccattttacggattcctcagatttaaaaatgtctcagatagatatttccaaattctatttctattagcctctgtggataaagagttcctgaaactctggttttactttttttggaaaaaaaaaaaaaaaaaaaaaaaaaaaacaactcccaggaaaatgaacactatattgccaagctgcctccagggaaaggttgaagactagttaaaataattctaagcgtattgaaaaaagaaagtgtaaagatccagtattaaaatgaatgtttgagaatacagtggggacaactaggtaattcactgtcttacgcttttcagaagactggccctttgaaacgcagcctgttattgttggtcagatcatgtggcacttaagtagccccttggtcatatttttaaaagcaaatatagacagtgacagtcctacaggggaaaatcacagatacattcatatgcacctcttttgttcttcagatattgagtgggtcagctaaacaagatcactttgaatatgaacctctttgtattagtcacaccaacaaaaaagtttcaaaaaaagttttcactttcctacatttgctaagtctgagctttaaaaaattctaaaatcctctaaagacaatactgaagctgataatataaaaagcaaattagagcactaatgattattactagatgcaccagattaactgcagcaggttggtgatgggtgatataagcaaagacataatatttcaatcaactcatgatcataggcagattcaaaagttaaaatgaatataatgtaatatatatttcaatatagagttgttatatataatgtgtatgtcctaggtttcagaaatactgcaatgtagtgtattgtagttaagtaagcatacctaaatagtaactcatattctttcacaaagtcactagtactgttaattaaaggaaaaaataaaaccgaaacaactaattgtttttccagtaaaaagaaatacctatggttacagttacagacttcttttggatatagaaagacaatatacattttaaaaagtaataacgacaaaaaagttgcaactgtaagtagccttacttaacaggggaaggggaaaagtcaccagaatagaagaggaaagaaaatgtcctctgacttctgtaaaacagaaataatgtacaaatcataaaaaataacaaaccatctagtaaaagaagggcatgggagtgagaaaactgaatcctgaattccaggccaccaaaccctcagagtccattcattcagtatattatactagagtggcattctacttcaatgcttgagatgggcaagagcaatcaattcctacagattaccaaaaaacattccccccaacagtctattggtttgctagacatggtaaacaacccactcctggaaagactttggcaaaggccacattggtttcaggagacacagtttgtgaattacgatgatatcttgtgagtacaggcagaattaggaagctttagtttgagaataaaatttatgtgtgtgtgtgtgtgtgtgtgtgtgtgtgtgcacactgcattgcatagaggaaaggaatgaagacctttgagctatgggatggctcaggccaaagtttgtgtgggctttgcctgcctggcattggtccccacccctgccacctccaggagacctggggagacgccctggactgctgctccctcttgtctgctcaccagttgaagacttctgttataccttattatggaggaaaacagcctgtccctgtgggtttgctgtggattcaacaagctgcatttgtttctcccaattctgaaacattacaaaaagcaacagagtgggcaggtgactgcttcctgggaagggagccacaagtcttaaacacaatggtgggaagaggcaactgtatctatgcacgaggacctctgcctgtgtgtgcttcctttggggggcacacacacttccagatgacaataagtatatacacaaacacacacatgtgcacacatgtcaataaatccaatagaactgtagagtttgttaaatgcactctactccacataagcatattcaagtttctcatgaaacggatacatagaaattactgatggttgggctccttcagaatgccctaaagtctcatcacagatactgatgcacccaactaaggcaacaaagcataagcagatacgtgagatatgtcagaccttcgacttctaaccagaagttcaaaaatgtatcttgttgtcactgggcaatatgaatgtgaaacagttttgtgctgagggaagctcacactgtgtgtgcacatgtataaataatgtatactcatttatagacattttggacagcagcggtgacatactggatgggttaagactctttcattattagaatctacatataaattgcaatgagtttgctgggtaaaaacaactgttgcaacactagtagaaacagatgcccccaaggtttttttttttttttttttttttttctctcttggatgtatcaaaatctcattgaggcattctaaaccaaagaaacctctgaatttgaaacagggttagtagggacttttatacccagctgggcatcccagaagcctggactctcaggactgtggctagattttgcccatgatctgtagattatgctcttgcaccggagacttgaaagttatgagtttgcattcaaacaaagaaccaccagataaaacagatgttctctaaaactgaggaaaaaaagtttagagatatacactgtatagagaaagaaagctttttgctggattgttctccttgttaaggaaatgtttaaaactagtactcccgggcacctgtgattgcattttataggattctatttagtaatatgatgtctattttacattcagccccaacctacgtcactgaaatagaataggaaatagcagccactatctgagagtacccagttctaggaaagtttggtgcctcctcaagaagtcactatttccatagtcctcaatcatgaatagggcttgtttttgtgataatgtaactattaaacagcaagaaatgcctataacttcagagccttctcatttctatatcttttatcctcttcccagggctttctgatttaaggcaataatgctacactataagtagccttttgtgaaaataccttaattgaggtcacttaagattagatttcagtctgaaagtctacagtttacggagcaaaaggtggagcctaaagaaaccactggcaggtgttttagtcagtggtgtggaaagataatgtttcttgtttcaacccagggcatttttacccatcatgcagtgaggagaaaatacatagttctgaaaaagaacccacactaggtagccctaattttctatctcttcactctaaaaaggatggaaacaagccctactgttccataaccattcccagggatcggctaaggtacattgctgactgctatagactcagtgttcaaggagaaaaaaatcttcagagacttagaaaactctttgcaatattttggtcaggctgatcgtcttgatactcagtgctagaaatgatgctttggattagtagtttccacattctgaatttataggaacactgagtcaccacagccttttttcttgtaaaggtttaagtgatatcagaaatagcaactctacacggaaagcccttgggaatatgaaaatactctctctcaagagcaagggctcttccgtgccccttttctgcctctgtatgtagcctgagcaccagggtagagattgcttttgaaagtttgccccatgtaatctatttcctggctacctaagagaacagccgttttcttcatgaaaacacaaagaggggaaagaggctgctgctgttccagtgggaagttatgtctagccccagaaggcctggtggctgggtcagctcaagcactctcttcatgcactgcaggctcaggaggcattgggttgctttgctttttctatggaattagggagcctattgaaattctagtgcacccctccttttgtttgtcaccaagtcacatggttctgtcttcagtatcctatttttctttttttttaatttctttttctgaggaacaaaattggccatttaaataaagttcttttctagtgagtaaagaggtttctcagagccagaaatcactgaaaagagagtctgtcgaccctgcccatggaaaagcccagagatttctctaaccacttcttgccaaacttcctagttttgtgattggatgtttcttggtttagcattgtttggtgctgaatacattttgcaattcttttgttctctgccctagagcttccattaccctggacttcaactcattaccaaattaaagaattcttttagaagatttcttttaagagtcaggtcacaacagaaagggcgccctcctgttctcctaaatctcaagggcatctcaggttgtgtctgctcttacgttgcaccttccttttgttcccttttaatgcagcagcacactggctatagcagaggcagacctgatttgattatctgataccttttccacaaaatcatatatcccctgctcccagccccaactaatcaaataacatcttctagaacaacagaggaaagctccagaatgggtgtatatcctgtgactcctggccagatccaccttgctccctgtcttcctaggggtcacaggtgttgggagcattgtggaggagccccaacaaggaagcaacatatggctttattatgttttctcaggaatcgaaggggttttataaggggcatatctcatttttgacttctgtgctgagagaaaatattgagttttgggcgcaggcagagcacagacaggacagctggtgttcctgtgtgagggaagtacacatagctcaaggctttaggactgaatgtgaaacaaacatacctggaggaaaacttttttcattatcagaattcacaaattcttactgttcatgggttgaaaaagagtatttgggaccttatagaatattttgatgatacaaaataaaacccttatgacttttaaacacagcaaacccaagtctttctaaggccaagagctactatgatctctaagatgactaggaatgaactgaggctagaatatgagcaggaaattatccagcacacttaatcatggcacaaatagattcaaagcattaggaatttgggaagagaacggtctataaaactgttattaggagctaaagtttacctctcaattaaaagatacaggaaaccattttgatacagagattttcatttcagattttttttctttgcttagcttgtttccccctgtgtagaattgtaacagatccatgtgttccaattattttcttttttaggattatatttcacacatttgggggccttttttgtacaaatattggcatgtaataaggaaaaattgcccatgatgctgagataataccagtgtttttagtggtagaaaatattatttttttataaaccatatctaaatatcttgagataaaaattcccctttgactttttttcctctcccttgtttggcaaattccattttaaaattataaattgctaaaaaatgtcctttccatactatttctctcttccttgtactcatcctaagaagtcttaaatctggaacatttgcttttatcttatctatctgtttcctggctactagaaagaaatttttttagcactcatatcaccctaccatgaaggtctaaatgtaagatgactgtaggacttgaaacaaaaaaaaattaaaaagatccacactcattctttgattttgaagcaaatgtctttccctatttctaaagatatttgtgattgtttaacttaaaagtgagaattgacaatctaaaagcatctctatccttttgaaacaggtccagattggtttatttcctaaaatgtgggtcagtttggaaagtggccatttgatgggccaggaacatagcaataaacaactacctctttgctcctccagattagatctcccactccaatccagcttcttcctctttccacaaaataatttgtcaactattttagaatgtgacatatttgggaaggataaatgtacagtaggaatatgtctactgctatgcaaacctggctggtccattttgtcatggactacaatgattatatcacctcattaagaattctttagggatcctccacctcctcccccactcccttttttttaagagacacttcctttacagggaaaggatgatagactcctcagggtttcaagtcacctgcagctttttctctacatgttctaccaaaagaaaaggtggattctaacccaattgcttagcattttacatggcaaatcagcattaaggcaaatgggtctctctcagatttgagaaacagaaagctacacgtggcccataatggcacctaagatcaacttttcaggcggtattagtgaaaattcttcctactttgctaaatttgaacaaagacactttcaaatctactgtgaaacagtttaaaatattttaaagtggcttttggccttctttcatttgtaacatgtattgagtgatttcatgtcattgtctcctagctttaagagtttttttcttaaggtcaatcttctcttttcattttatgggtggaatcacttgttttccaaaatatcaaaacaattccatgacatagttaattaatgctccctctattggtggtaagtggaaatattagtcttacaacactgctattttaaaaagcaaaattagcaatagaaaaatgaacttactttatctcggaagctgttcctcactaactgttaaaacagatcagttttggacatacagttcttggcaggactcctcttagaaatcacaataggttacacttaatagtcagttaaccacccaagtttacattaaaacttctagcaaaatatccactgaattaagcactgtgggaccaaatcaaactcacaaacacttcagttacactaaccttacaaagcatcacaaagaacttatgaaaaagatccaagttaaccaaatgtctaaaatatatgaataaaaccaatttagtcattacagagttgtttgtgttggaagattttccctcgtttgctgcacagtttttgtaaataaaatgctgacaggaaaattagaaggaaaattaaattaaaatgtaatgtaattttgaaactaaaatacgctctcctttcttctttttaaaactgtagtttggtgttttgctttgtttaaagatttgctttcccctaagtatgttaaaatatgcccagcaatgaaatcactttgggagtttcagctaggtttaagaattcctatatttgagctggaatcccttcaggacactgtctataatgaaaatgtctctattataacaccttgatcaggaccgaggagagaaatccctactaggaagagagagtggcatctggtatgatgcaatagattggtggtcttttgaatggtggctgttggcatctgggaatttttttgttaatttccctaaaacctttcgaagaagcaagggttaattcgtcatctaaagaatgatcatcttattcagccctcttaaccatggtggaaacagtcagaaggtgatatttggaaggaaaaaagtaattttggcatcaatgcatcttgatctataacaggcttctcataatgatgctctttgtagttgggaagggtgaggagctatggcagagttttgtgaactcctcttcctggctgatcacaaaagaaaagaccccatttatcaagacttctagactattagtgtttcactaagaaaaaaagtaaagtcaatagaaattctagaattgtaagatctcaatgaaattttggagaagcaagcaatctctttctgaaagataaagtctcttccatgaaaaagaacagaattctagatgaatcagttgaaaaaattattcagtggggcaacttaagcttgctaaagtcaaagaactacatatcaaaatacaaagcagcaattcaaattacagcagggatgggctggccacagaggccctcatcaacccaggcaatacttaaaataataaaaattaagaaaaattaaaaaaaatatgaagaaaatatccttcctctctttcaaatataactttagttgccttttattctttctatctggaagcagtatcgctaaccttaacagtcttgacttaccaaaaaatatatatatgtgtgtgaaataaaataaaagagaaggaattggtggcagtgtatgcaaaaccaaaatgaaaaaaattacttttaacaatttcactttttttgtttttttttttacacaaatactgttgtaaatatattaaaaaaatcagcattctatctggtaaacgtcacttttgcccctctataaaattttgaattaaaaaagcctcaagaactttttattgttccccccaccctccatttctttttctttttctcttccacaagaatatatcctgacactttttttttttttgcaaagattgttggaaataatccttctcttgtacctagaaacataggtgcaaatttctgatatctttgttttatctgcattcctgcctttcatgaaagtccctcttgattgtgctgaggctgtggctcagcgaagacactgaataaatacgatagccactgttgcttgttgcttgtccaagtcttcctggcttctgctgcaagagggggatatggagaaggtgggccagggtgtgtggacccgggcagaatctggggaagaagcctgccattcgtctttctttcccacaccaccgaacccactgcccttcccacccccacagcccttttatgaaatcagacaacgtggtaggtggaaaacagcagggcctttcctctgggttttcaaccagaagtgatattccacagttttaactggttactgtgaagtccaagcggccagaattgtgaaaatgtccactgaaacactgcaagcggtgtacttaaagacagtaggccttttagattttgttatatattttttgtagtgctcttcacaagtggaaattttttttttttttttacttttttttaaaagatttttttgtaaagaagggttgtatttagaggccagtagctagagatccaaccagtggacctcttgaagcactaccaggccttaaggccaccatccgagggagactgggaaaactattattcacccaagcctccggaaatgtaatgtaccagcaggcaaaaaacagttcttcatgtagtacaaaatgaaacgaaacaaaaacaaaaacagaaagtaaaaatgaaaccaaaacatttcttaaattctagtgccatagcttttttgtttgtttgttttttgttgttgttttgttttgttcataagaaagagagaaagatactacttatccgtcagacacatgcatcctcatgtggtcgttgaactgctcgatttggtcaaactttgctgggcagacggagcagacgtaagtggtcccctccgtgcaggccaccacgcctggggggccagcgcgggcacctgggggtgtgcctgcagggggggtcccattgctggcactgtgcagggccacgtgtcgctccaggagggtcttgtgagagaacttctttttgcagatgtagcactcgtaggacttctctccccggtggaggcgcatgtgcacgttgagggagctcttctgggtgaagcgcttgttgcagatactacactggtatgccctcactcctgtgtgtgtcaccatgtgcttgataaggtaatcctttaaggagaaggagcgccaacagatgctgcattggtggggcttctcacctgtgtgtacgaacatgtgcttgacgtagttctgtttggcggtgaaagtcttgttgcagagagtgcactcataaggctttttttcgccttgcccactggctgtgctgtggcctgcggatgaggccaggggctgtggcgctggcagctgtgcagtaaaggtcgacagaccgggctgggacactgtcacaaactgggtctgctggcctgccaggggctgtggcaggctgaagaggaaaggcttggggccactgcccgcgggctgggtagtgaagagggctggcaggtaggtgttgccagctgtgccaatgacctgcgtgttgctggtcaaggtcagaggcatcctcaggttgctggtgagggtttctgtctggcgtaagtagagctgggtacttggcaatggctgcccgatggacgtgttgaccgaaggctgttgtaggacgctcttgtcggagctgttgctgacagtgataacagtgctgtccatctccacttcattgcttctctccggagaggaagcacctgtttctagctggtttgtctgcggaccaccctcagcgggggcttctgcagcctgctcgggttgggtgggttcagcctggctgtcccgcgccgccccaggcccaaactgctgctccaccgagtcaggctcggtgcctatggaggagctgacgcccgagtcgaagctttcacctttgggctcactctcggtgccctcggcctggtctgtgtcttccgtgcactcctcggattcgttgcgttccaggatctgcaccctttgctgcccgtagtagtcgtaatcgtcctccatctcctgcttgatgtggatgttgcccactagggtctggatgcgcacaggccggggctgcttgcggcagtgcgtggtctcgggggtggtggacaggtagcgctccatctgctgcgagcgctcatggatgcgtgtgatccagctggggtcttccatgtggtggtcgcggggcaggccgagcgcagtctcgtggtggctgaccactgcgccgctgtaaaaagagcgctcgccgctgccattctgcatggagcacgcgtagagtgccgagtagatcctgtccacgctgtgctgtgggtggctctgcaggtagcccgactccgtgtcgctgctctggcctgacgtgcctgactcgggagtgccccgcggcgtgtcctggcccgagtcctggatccccgggaacacatcgcccacgttctgtgacacgatgcgcgtgcactcgtcgatgactgttttgatctgcaggatgctggcggccgtgaggatctgcagagcttccgactgcgagacccgtagcacgccgctgtacatgaagtcaatgagcttttgcactgactgcactgacaccaccgacgggatctcgatgtcgctgtagccaagcagcagtttgtcctggaagaaggggctgccggctgccagcacgcagcggtgtgcgcgcagcatgctcccgtggatgcgcaccgttacgtcacagaagtggccacggttgcgctgctcgttgagggtctcgagcacggaattgctgaagttgtgaaggttgatgctgtgaatgcgctcggtcatccccttgcaactgatgtcacaatcagatgacccggtgtgagcgtgagagtttgtcagtgaatgtgttgagtggatgagggctgggtctggagacaaaacagcttcaaagttcaggcagggaaggcccggcttggcgctggatccacccggctgagtaatctcattctcctcagatgccttctggttttcagctgtcttgggtttcttccgttctagcatttgtcaggaagcttagagacaggactcgtggagtaatgggaggagcactggactgggagtcaggagacttgagctaccgtactagctgtgcctctaacttgctgtgtggccttgggcacctcacttcacctctctgggcttcagtttcctcatctgaagcctaagagggatgttagtctcccaggtttagcgttttccagtaacatagaagtagtagtttcaaaatcaatggtgtcactcttcaggtaaattactccaaggcttgggcctagtgcagatgttcattggggcagggagcagagagcggctgcatgtaaagagaaggggcaggtcacagactgatggtcaaagatatgaattaacagaatcaacaggtgatttggtatcagtactgctattggctggcgggtttcacctcagacagcaatgtcatgaggaatatcctgttagtaatgatgaaacattaggaatacagtgcagctcaatcttttgtttttaaggtgcagtgatttcagtctctaaatgtaacttcaggcagtctgtgcagctatggggcacaaacttgcaattcatcaattcttcagccttcagagtcccaaaggcaattcttaacacttctttttatttgtagtggcatggatgacggagcagaaatagagaattcttgattaaccaggagaagaatatcataggcatgggtgtgagatcaactggagattcaaggaagctaaagtgcccagaatgaactaatgttgtaatgtagactgtgagcagagataaaattccagaagccaaggagtgttgtacggtaagtcctggcagtgcctcctcgcgctctttaatcttctttcctcaactcctaaacttccccccgcccctacttcttcggcagaag

SEQ ID NO: 16694 - RNA, 213 nt, Homo sapiens
  source 1..213: mol_type = other RNA
taaaatttgcatccaggacggtcggaagaggcgccttcccgtcggaggcgaggcgcgggcgcgtgggagctttctcgtgtgcgctcctccctgtcctccgcctgcggccggggcgcagagtccgtggtcatatgagaatgacagttttttgtctgtttgttttggcgggggcgagggtggctgcctctttctttcttttgcccgttcgagggt

SEQ ID NO: 16695 - RNA, 466 nt, Homo sapiens
  source 1..466: mol_type = other RNA
taaagagccctgtggagacaaagaagcgtgagagactgacaggaatgacaggcagtccccatcacctcccagctagcagccacacctccccgtacccagtgtatccaagactccgggccagctgcgtggcctggaggccccgcttgcccatctgacagaagaaaacgagatgctcatcttccagctttggcttctcagcagaatataaagcctggaaggcagctggctccatctgcagagcactctccaactcggacaccgggatgttgagcgcccctgggatggtcccagctgccgcctcctcgcgagagcgcacgtcgaagagccgggcccgtccggaggctaggagtgaacggagttcaggaagcgagaccgtgggcgctccagccatggtgcgcgtagcaaccgcgagtctccggagtgcggccctggcccgccctctcggcgcctgcaacatctcccgttc

SEQ ID NO: 16696 - RNA, 76 nt, Homo sapiens
  source 1..76: mol_type = other RNA
taaagtaaatatgcaccaaaactgtatttaccaaaagtaattttggtgcatatttactttaagatgttactggagc

SEQ ID NO: 16697 - RNA, 337 nt, Homo sapiens
  source 1..337: mol_type = other RNA
taaagtaaatatgcaccaaaattcagctcctgtaacatggccgcctcggagttcctgcgaatcttctccacttttgagtctggacgaatccatggagaaagctttcccacaattagcgtattccagtccctgcttctccgggatgactagtctgcccttctccgtccccgagttcggaccccgcattccgctcgtggaggtccggccctcacccctgcttggccacagcccctagtgtgtcagctatttcggggacgcaattcaggtccctcccgctggacacgcggctcccaccagcacccccgaccgccatcgccgccatctttctcctcgcgct

SEQ ID NO: 16698 - RNA, 456 nt, Homo sapiens
  source 1..456: mol_type = other RNA
taaagtaaatatgcaccaaaattcagctcctgtaacatggccgcctcggagttcctgcgaatcttctccacttttgagtctggacgaatccatggagaaagctttcccacaattagcgtattccagtcccttcctgacagcagtaggtctgatcgtgtctggggaccgggccgattcttagcaggttcctgaatgaactccctcttgaaacgcggatggaagacaggcatgcagaggaaatcaaacccctgcttctccgggatgactagtctgcccttctccgtccccgagttcggaccccgcattccgctcgtggaggtccggccctcacccctgcttggccacagcccctagtgtgtcagctatttcggggacgcaattcaggtccctcccgctggacacgcggctcccaccagcacccccgaccgccatcgccgccatctttctcctcgcgct

SEQ ID NO: 16699 - RNA, 371 nt, Homo sapiens
  source 1..371: mol_type = other RNA
taaagtaaatatgcaccaaaattcagctcctgtaacatggccgcctcggagttcctgcgaatcttctccacttttgagtctggacgaatccatggagaaagctttcccacaattagcgtattccagtcccttcctgacagcagtaggtctgatcgtgtctggggaccgggccgattcttagcaggttcctgaatgaactccctcttgaaacgcggatggaagacaggcatgcagaggaaatcaaacccctgcttggccacagcccctagtgtgtcagctatttcggggacgcaattcaggtccctcccgctggacacgcggctcccaccagcacccccgaccgccatcgccgccatctttctcctcgcgct

SEQ ID NO: 16700 - RNA, 387 nt, Homo sapiens
  source 1..387: mol_type = other RNA
taaagtaaatatgcaccaaaattcagctcctgtaacatggccgcctcggagttcctgcgaatcttctccacttttgagtctggacgaatccatggagaaagctttcccacaattagcgtattccagtcccttcctgacagcagtaggtctgatcgtgtctggggaccgggccgattcttagcaggttcctgaatgaactccctcttgaaacgcggatggaagacaggcatgcagaggaaatcaaacccctgcttggccacagcccctagtgtgtcagctatttcggggacgcaattcaggtccctcccgctggacacgcggctcccaccagcacccccgaccgccatcgccgccatctttctcctcgcgctgtccacgccgggattc

SEQ ID NO: 16701 - RNA, 5362 nt, Homo sapiens
  source 1..5362: mol_type = other RNA
taaagtgctgacagtgcagatttattagggaactccagtttttgccttcccctgaaaaacgtgactttgccagaagcataggtactgttctatgaccaattccagcctcaagaactataaaaatagaatcaatgttcatttttatcatctcgcctttgggtaccaattcagttgtgggagctattttttcagtttcatttgattcttcaagaaaccacatttttaaagtctttgtatccttcttttcccataaatgtgcagtagaagaagccgtttcttctgggatggtttccttagttgtatacagtgctgaagttatggtaatcatagtatttataataactggtgaaacctttagtgtcagggattttactgacatatcgatcacttgtggatctgtacctttctgagtagtttgataaaacaagtcacagggctgcaaaacagtagtgattttgccttttctcttgactggaagaaacgggcaggctctcacttggagatctttaatggcagcagtcattgtactattttcaaggttacctttatagcaaatttcacattgtgttgtaatgactaaagcaggagcatcattttttgtcatgtcagctacaaacacaatttcaggatttttaataataacattaatttcccacttcactgattcctgtgtaggtacttcttccttagcagtccatgtttgcacactggtttctacagcagtgcctgtggtgtaggcctcaagaaagacatttgcaacagtctgcagaaattctacgcttgcacaaatatacatttcttgaaagaccgcatcagtcacacaaccatctctgactttcctgtactttatatccatcatgtcttttttgtcaaaaccaactgtcagtcctatcattcgaggagttgctttcttgacatgaggtcttttatcatctaaaatacagttttttaatgagaaggaagaaaatgttgagccatctgtatacatttttaaagtacttataatattctccaatttaaattcagcaagtttcagagaaggatcacgaacatctgtaaaggaagcctgtttaggacctggactatacagcaccatggtgagatcatcagttttgaagcttatgtttagtgttgtcttaactagtaaggcacgtgaatgtacttctaccacagcagctgtcaccacagttgctcctcctgaatggtgtgaagcattagtagtaactccactagtggcactgtattggtcttttgttacagcaggtgaggcactaccatctttttcataccatatattgccatgcaatgttttaaaaatagttgttatatcttcttgactaagaatgaactccattggtttcagctgagcatttacattaaaacaaggaacttcctggtaccactcccagcataaatttcgttcaaccacaacctcaagatttaatggcaggagtagatccagtacttcctggtatgcatcattaataaatcgagatctgtatagtcgcatttcactcagctttattgttatcaaatcaataacaggtgggggagagctctggctctctgttatcatatgaaaggtatttgtcattgtaattagtccaaaatcagcaacaaaaacattttcagaaactggagactgcgggatgaccacaactggggctttgatgttaatatccagtgccattctggaactcctttgtgcgagttcttttacaccagtagcagccattccagctgcctgaacagttgcctcagccaaggcttgtttagctgcctgaaaattatctataaaagccaatatagaatatagaaatttcgtgacaaaaactacttcaatgcaaccaactattaaattaacctgaatgtcaaccacattcatatctgtgtatgcagaaccagcagttgcatccatgtaagaaaccattttgaagctgaaaacttcttttccagtgatataaacagcctttttgtatatagctgttatatcagaatctaaaacaattatattccttagctttgcgtttatttcagtttctgaaggcctcataatcatctcagaatcaagccctaattttttaatgacatctcctttgtcttcagtctctgtagtggacactggggctgatttttcctctgattgcggaaggatattatgaagataatttattgtattcagaagtgcttcagtgtgtaaatgaatatccaaagaggaaaaatttaccttaatcaattgtaaaacattgttataggtacttttcaagtcgggtacattcttttcagcctttacatattccagcgttaacaggtcttccattgtgttatccagggttgtaaccaaataaactggtttcttgttttcatccaagtattctgggcattttaagcagaactctttcaaaaaggcatttgctttcaaatcgtatgttctaatctcaatttctgcacccaatcctaaaacaagaatttctaccacagatagttcacaatctccaacaaggtgataaaactcgatcaaaacctttggtacttcaaatcttattttaaatgtagtcatatttactgaacaatcctgcttttgtaactttctggttcgaatacttttaactccagttggaaactgaagaggttcttccaagggactacatggtgcatcaaaaaattcctcctctgaatcatcttcagaaacagatggaagttccaagagaggaattattttctgtgaaatctgtgatgttcccaaagaagtagatgtttgaatctggaatgatttgacaggggcagatacttcagttactggttcaggttttggaatgctttcaatcaattccataatcccttgtagttttttatctgagattcgtaaagaaataagaggtaactttccataaatcttgaatttgggcatccttacatccatgaaaaccatggccttagacagttccaaattgaagtgcatgggtaccaaaatatgctgggtagatacactgagttttcgtgcttctctccaattatcaccaactctactgtaaagcagctgtacacttgtaagttgaatatcaaatgaatcataagctctatccattatctctttaagattggcctcaccttgtttcacatctggtaattcagaacgacttttactcgtcacctttagatgaccaaggtccaaaagaagcagatttgatgtaggactaaaaattccatcttgtgggacaataatatatgaagccttcaaattaattttgagatcaagaactttctgtgtttcaataatatacagtagacctgttgctgtcttactgcgaaattcttccagttttgtcaaagttgctgcagtgagctgtgctagatgtacctcttttggaggtctgaagaattccactatactattcactgtccttgcatcatatatgatttctaaaggttcagcttctatgatacacctctgagaaacagtttcatctaatggatttatctcaaatgtaatttggaaaagtgacattgcatcatccaatgaagacaggaggcggggtttttctgaattatctggtaagccagtaatatgaaatgaatctattttagtttcaaattttattgcttgtgctcctggtctttgcacaattaaggtgctaaattcttctattacaatatctaccagctcaggtttttgatgattttctcttagaacaatagacatacttttcaagtggacaaaaaacttcaaggcttcaaatgtttttagtaaagttggatcaactgctgtttcactatagccaattgcttcatagagtaaagctttttcttcaggtgtcaacatttcttcaagagtttcaggttgaacatctggttgctgttcattagtattttgttctgaccaagaccatagccagctaaaccaccctttattatcctctggatcttttactccttctttgtaaattttgtatccagctttctttacctcaacttctgccgtctgtctagctatagttatattaaagacatccaaggttttttccaactcctccaaagacacgagaagttcaccaggtggcttcttacttgttaacttttttttatacagttctttatattgcttcactttttgcctatgttttctaatatgcttccatgaccacatccataacctggggcaaacatttacttcaagaacgccatgtatagcataagcccaccattctctggcatggtggtgaagaggcacatcaggtttgaacttcctatatggcagattttgtgccatcatatcaactgattcaagaagctccataatactgaaatactgtggtttattaaattcaattgctatgttatgtaactcaatttccaagtttattttgggggcagaaaagtcaaaatcagatcggcgattcatcacaagtttggcattagcagatatgggacgaaatacaaaatcataaccttctggaacaatattttcattgacaatgccattcttcaagtcgtccaaggagttatcataatcactaagataaaacatctgagacttcacattccaataggcaaacaggttatccaatcggattaacttacgaaccagtttctcagtttcatcatgtaaacatggaacccagtattgatcagttgtctgcatgctcagattttgaagggaaataccaaatgacagcggtttgtcccgatttgtgatatcatcttcataacgaatatggatactggaaattttcacctgaagattttttatgatctgtgtaactaatttttctgcaaaagtgtcctgtttttccggcagatgttgttcttgatcaactactttttgttttgcttcttctattcttttcagttcctgttgctttgcttccatgagttgtttctcttcttttaaaggatcatattttattctagaagaaggcactataagtaaataaatttcttccaatacggcttcaacaggttgagtataaaggtttttccatggaattataagtttaagattacctatgtgaccaactttaactttaaatggtacatccagttgactcagggcattttctttaatttgaagattcttgagggccacagctcctttccagatgcccagagagagctgggacgtgtccaagtccaccacatagtcccccaagaaccggttcaacacgtccacgaccaccgactcgaaaaccatgttcctcagccgtggtgggcacggcagccggcccgtgcgctcctcctcccgccgccttccccacgcccctccctcgaggtaattcggttcaccggctccggggcggcttcagctgcggcgcccccgctggcccaacgcgcagccctagcgagcccagcgagagacggaggc

SEQ ID NO: 16702 - RNA, 5479 nt, Homo sapiens
  source 1..5479: mol_type = other RNA
taaagtgctgacagtgcagatttattagggaactccagtttttgccttcccctgaaaaacgtgactttgccagaagcataggtactgttctatgaccaattccagcctcaagaactataaaaatagaatcaatgttcatttttatcatctcgcctttgggtaccaattcagttgtgggagctattttttcagtttcatttgattcttcaagaaaccacatttttaaagtctttgtatccttcttttcccataaatgtgcagtagaagaagccgtttcttctgggatggtttccttagttgtatacagtgctgaagttatggtaatcatagtatttataataactggtgaaacctttagtgtcagggattttactgacatatcgatcacttgtggatctgtacctttctgagtagtttgataaaacaagtcacagggctgcaaaacagtagtgattttgccttttctcttgactggaagaaacgggcaggctctcacttggagatctttaatggcagcagtcattgtactattttcaaggttacctttatagcaaatttcacattgtgttgtaatgactaaagcaggagcatcattttttgtcatgtcagctacaaacacaatttcaggatttttaataataacattaatttcccacttcactgattcctgtgtaggtacttcttccttagcagtccatgtttgcacactggtttctacagcagtgcctgtggtgtaggcctcaagaaagacatttgcaacagtctgcagaaattctacgcttgcacaaatatacatttcttgaaagaccgcatcagtcacacaaccatctctgactttcctgtactttatatccatcatgtcttttttgtcaaaaccaactgtcagtcctatcattcgaggagttgctttcttgacatgaggtcttttatcatctaaaatacagttttttaatgagaaggaagaaaatgttgagccatctgtatacatttttaaagtacttataatattctccaatttaaattcagcaagtttcagagaaggatcacgaacatctgtaaaggaagcctgtttaggacctggactatacagcaccatggtgagatcatcagttttgaagcttatgtttagtgttgtcttaactagtaaggcacgtgaatgtacttctaccacagcagctgtcaccacagttgctcctcctgaatggtgtgaagcattagtagtaactccactagtggcactgtattggtcttttgttacagcaggtgaggcactaccatctttttcataccatatattgccatgcaatgttttaaaaatagttgttatatcttcttgactaagaatgaactccattggtttcagctgagcatttacattaaaacaaggaacttcctggtaccactcccagcataaatttcgttcaaccacaacctcaagatttaatggcaggagtagatccagtacttcctggtatgcatcattaataaatcgagatctgtatagtcgcatttcactcagctttattgttatcaaatcaataacaggtgggggagagctctggctctctgttatcatatgaaaggtatttgtcattgtaattagtccaaaatcagcaacaaaaacattttcagaaactggagactgcgggatgaccacaactggggctttgatgttaatatccagtgccattctggaactcctttgtgcgagttcttttacaccagtagcagccattccagctgcctgaacagttgcctcagccaaggcttgtttagctgcctgaaaattatctataaaagccaatatagaatatagaaatttcgtgacaaaaactacttcaatgcaaccaactattaaattaacctgaatgtcaaccacattcatatctgtgtatgcagaaccagcagttgcatccatgtaagaaaccattttgaagctgaaaacttcttttccagtgatataaacagcctttttgtatatagctgttatatcagaatctaaaacaattatattccttagctttgcgtttatttcagtttctgaaggcctcataatcatctcagaatcaagcccttcaatcttaatttcagaaatgttacatttctgatcttgaataaagatctgtaaacacgataattctgctaaaatctgcaaagtaatgatatcttcatttgtggatagttttaaagctaattttttaatgacatctcctttgtcttcagtctctgtagtggacactggggctgatttttcctctgattgcggaaggatattatgaagataatttattgtattcagaagtgcttcagtgtgtaaatgaatatccaaagaggaaaaatttaccttaatcaattgtaaaacattgttataggtacttttcaagtcgggtacattcttttcagcctttacatattccagcgttaacaggtcttccattgtgttatccagggttgtaaccaaataaactggtttcttgttttcatccaagtattctgggcattttaagcagaactctttcaaaaaggcatttgctttcaaatcgtatgttctaatctcaatttctgcacccaatcctaaaacaagaatttctaccacagatagttcacaatctccaacaaggtgataaaactcgatcaaaacctttggtacttcaaatcttattttaaatgtagtcatatttactgaacaatcctgcttttgtaactttctggttcgaatacttttaactccagttggaaactgaagaggttcttccaagggactacatggtgcatcaaaaaattcctcctctgaatcatcttcagaaacagatggaagttccaagagaggaattattttctgtgaaatctgtgatgttcccaaagaagtagatgtttgaatctggaatgatttgacaggggcagatacttcagttactggttcaggttttggaatgctttcaatcaattccataatcccttgtagttttttatctgagattcgtaaagaaataagaggtaactttccataaatcttgaatttgggcatccttacatccatgaaaaccatggccttagacagttccaaattgaagtgcatgggtaccaaaatatgctgggtagatacactgagttttcgtgcttctctccaattatcaccaactctactgtaaagcagctgtacacttgtaagttgaatatcaaatgaatcataagctctatccattatctctttaagattggcctcaccttgtttcacatctggtaattcagaacgacttttactcgtcacctttagatgaccaaggtccaaaagaagcagatttgatgtaggactaaaaattccatcttgtgggacaataatatatgaagccttcaaattaattttgagatcaagaactttctgtgtttcaataatatacagtagacctgttgctgtcttactgcgaaattcttccagttttgtcaaagttgctgcagtgagctgtgctagatgtacctcttttggaggtctgaagaattccactatactattcactgtccttgcatcatatatgatttctaaaggttcagcttctatgatacacctctgagaaacagtttcatctaatggatttatctcaaatgtaatttggaaaagtgacattgcatcatccaatgaagacaggaggcggggtttttctgaattatctggtaagccagtaatatgaaatgaatctattttagtttcaaattttattgcttgtgctcctggtctttgcacaattaaggtgctaaattcttctattacaatatctaccagctcaggtttttgatgattttctcttagaacaatagacatacttttcaagtggacaaaaaacttcaaggcttcaaatgtttttagtaaagttggatcaactgctgtttcactatagccaattgcttcatagagtaaagctttttcttcaggtgtcaacatttcttcaagagtttcaggttgaacatctggttgctgttcattagtattttgttctgaccaagaccatagccagctaaaccaccctttattatcctctggatcttttactccttctttgtaaattttgtatccagctttctttacctcaacttctgccgtctgtctagctatagttatattaaagacatccaaggttttttccaactcctccaaagacacgagaagttcaccaggtggcttcttacttgttaacttttttttatacagttctttatattgcttcactttttgcctatgttttctaatatgcttccatgaccacatccataacctggggcaaacatttacttcaagaacgccatgtatagcataagcccaccattctctggcatggtggtgaagaggcacatcaggtttgaacttcctatatggcagattttgtgccatcatatcaactgattcaagaagctccataatactgaaatactgtggtttattaaattcaattgctatgttatgtaactcaatttccaagtttattttgggggcagaaaagtcaaaatcagatcggcgattcatcacaagtttggcattagcagatatgggacgaaatacaaaatcataaccttctggaacaatattttcattgacaatgccattcttcaagtcgtccaaggagttatcataatcactaagataaaacatctgagacttcacattccaataggcaaacaggttatccaatcggattaacttacgaaccagtttctcagtttcatcatgtaaacatggaacccagtattgatcagttgtctgcatgctcagattttgaagggaaataccaaatgacagcggtttgtcccgatttgtgatatcatcttcataacgaatatggatactggaaattttcacctgaagattttttatgatctgtgtaactaatttttctgcaaaagtgtcctgtttttccggcagatgttgttcttgatcaactactttttgttttgcttcttctattcttttcagttcctgttgctttgcttccatgagttgtttctcttcttttaaaggatcatattttattctagaagaaggcactataagtaaataaatttcttccaatacggcttcaacaggttgagtataaaggtttttccatggaattataagtttaagattacctatgtgaccaactttaactttaaatggtacatccagttgactcagggcattttctttaatttgaagattcttgagggccacagctcctttccagatgcccagagagagctgggacgtgtccaagtccaccacatagtcccccaagaaccggttcaacacgtccacgaccaccgactcgaaaaccatgttcctcagccgtggtgggcacggcagccggcccgtgcgctcctcctcccgccgccttccccacgcccctccctcgaggtaattcggttcaccggctccggggcggcttcagctgcggcgcccccgctggcccaacgcgcagccctagcgagcccagcgagagacggaggc

SEQ ID NO: 16703 - RNA, 5660 nt, Homo sapiens
  source 1..5660: mol_type = other RNA
taaagtgctgacagtgcagatttattagggaactccagtttttgccttcccctgaaaaacgtgactttgccagaagcataggtactgttctatgaccaattccagcctcaagaactataaaaatagaatcaatgttcatttttatcatctcgcctttgggtaccaattcagttgtgggagctattttttcagtttcatttgattcttcaagaaaccacatttttaaagtctttgtatccttcttttcccataaatgtgcagtagaagaagccgtttcttctgggatggtttccttagttgtatacagtgctgaagttatggtaatcatagtatttataataactggtgaaacctttagtgtcagggattttactgacatatcgatcacttgtggatctgtacctttctgagtagtttgataaaacaagtcacagggctgcaaaacagtagtgattttgccttttctcttgactggaagaaacgggcaggctctcacttggagatctttaatggcagcagtcattgtactattttcaaggttacctttatagcaaatttcacattgtgttgtaatgactaaagcaggagcatcattttttgtcatgtcagctacaaacacaatttcaggatttttaataataacattaatttcccacttcactgattcctgtgtaggtacttcttccttagcagtccatgtttgcacactggtttctacagcagtgcctgtggtgtaggcctcaagaaagacatttgcaacagtctgcagaaattctacgcttgcacaaatatacatttcttgaaagaccgcatcagtcacacaaccatctctgactttcctgtactttatatccatcatgtcttttttgtcaaaaccaactgtcagtcctatcattcgaggagttgctttcttgacatgaggtcttttatcatctaaaatacagttttttaatgagaaggaagaaaatgttgagccatctgtatacatttttaaagtacttataatattctccaatttaaattcagcaagtttcagagaaggatcacgaacatctgtaaaggaagcctgtttaggacctggactatacagcaccatggtgagatcatcagttttgaagcttatgtttagtgttgtcttaactagtaaggcacgtgaatgtacttctaccacagcagctgtcaccacagttgctcctcctgaatggtgtgaagcattagtagtaactccactagtggcactgtattggtcttttgttacagcaggtgaggcactaccatctttttcataccatatattgccatgcaatgttttaaaaatagttgttatatcttcttgactaagaatgaactccattggtttcagctgagcatttacattaaaacaaggaacttcctggtaccactcccagcataaatttcgttcaaccacaacctcaagatttaatggcaggagtagatccagtacttcctggtatgcatcattaataaatcgagatctgtatagtcgcatttcactcagctttattgttatcaaatcaataacaggtgggggagagctctggctctctgttatcatatgaaaggtatttgtcattgtaattagtccaaaatcagcaacaaaaacattttcagaaactggagactgcgggatgaccacaactggggctttgatgttaatatccagtgccattctggaactcctttgtgcgagttcttttacaccagtagcagccattccagctgcctgaacagttgcctcagccaaggcttgtttagctgcctgaaaattatctataaaagccaatatagaatatagaaatttcgtgacaaaaactacttcaatgcaaccaactattaaattaacctgaatgtcaaccacattcatatctgtgtatgcagaaccagcagttgcatccatgtaagaaaccattttgaagctgaaaacttcttttccagtgatataaacagcctttttgtatatagctgttatatcagaatctaaaacaattatattccttagctttgcgtttatttcagtttctgaaggcctcataatcatctcagaatcaagcccttcaatcttaatttcagaaatgttacatttctgatcttgaataaagatctgtaaacacgataattctgctaaaatctgcaaagtaatgatatcttcatttgtggatagttttaaagctaattttttaatgacatctcctttgtcttcagtctctgtagtggacactggggctgatttttcctctgattgcggaaggatattatgaagataatttattgtattcagaagtgcttcagtgtgtaaatgaatatccaaagaggaaaaatttaccttaatcaattgtaaaacattgttataggtacttttcaagtcgggtacattcttttcagcctttacatattccagcgttaacaggtcttccattgtgttatccagggttgtaaccaaataaactggtttcttgttttcatccaagtattctgggcattttaagcagaactctttcaaaaaggcatttgctttcaaatcgtatgttctaatctcaatttctgcacccaatcctaaaacaagaatttctaccacagatagttcacaatctccaacaaggtgataaaactcgatcaaaacctttggtacttcaaatcttattttaaatgtagtcatatttactgaacaatcctgcttttgtaactttctggttcgaatacttttaactccagttggaaactgaagaggttcttccaagggactacatggtgcatcaaaaaattcctcctctgaatcatcttcagaaacagatggaagttccaagagaggaattattttctgtgaaatctgtgatgttcccaaagaagtagatgtttgaatctggaatgatttgacaggggcagatacttcagttactggttcaggttttggaatgctttcaatcaattccataatcccttgtagttttttatctgagattcgtaaagaaataagaggtaactttccataaatcttgaatttgggcatccttacatccatgaaaaccatggccttagacagttccaaattgaagtgcatgggtaccaaaatatgctgggtagatacactgagttttcgtgcttctctccaattatcaccaactctactgtaaagcagctgtacacttgtaagttgaatatcaaatgaatcataagctctatccattatctctttaagattggcctcaccttgtttcacatctggtaattcagaacgacttttactcgtcacctttagatgaccaaggtccaaaagaagcagatttgatgtaggactaaaaattccatcttgtgggacaataatatatgaagccttcaaattaattttgagatcaagaactttctgtgtttcaataatatacagtagacctgttgctgtcttactgcgaaattcttccagttttgtcaaagttgctgcagtgagctgtgctagatgtacctcttttggaggtctgaagaattccactatactattcactgtccttgcatcatatatgatttctaaaggttcagcttctatgatacacctctgagaaacagtttcatctaatggatttatctcaaatgtaatttggaaaagtgacattgcatcatccaatgaagacaggaggcggggtttttctgaattatctggtaagccagtaatatgaaatgaatctattttagtttcaaattttattgcttgtgctcctggtctttgcacaattaaggtgctaaattcttctattacaatatctaccagctcaggtttttgatgattttctcttagaacaatagacatacttttcaagtggacaaaaaacttcaaggcttcaaatgtttttagtaaagttggatcaactgctgtttcactatagccaattgcttcatagagtaaagctttttcttcaggtgtcaacatttcttcaagagtttcaggttgaacatctggttgctgttcattagtattttgttctgaccaagaccatagccagctaaaccaccctttattatcctctggatcttttactccttctttgtaaattttgtatccagctttctttacctcaacttctgccgtctgtctagctatagttatattaaagacatccaaggttttttccaactcctccaaagacacgagaagttcaccaggtggcttcttacttgttaacttttttttatacagttctttatattgcttcactttttgcctatgttttctaatatgcttccatgaccacatccataacctggggcaaacatttacttcaagaacgccatgtatagcataagcccaccattctctggcatggtggtgaagaggcacatcaggtttgaacttcctatatggcagattttgtgccatcatatcaactgattcaagaagctccataatactgaaatactgtggtttattaaattcaattgctatgttatgtaactcaatttccaagtttattttgggggcagaaaagtcaaaatcagatcggcgattcatcacaagtttggcattagcagatatgggacgaaatacaaaatcataaccttctggaacaatattttcattgacaatgccattcttcaagtcgtccaaggagttatcataatcactaagataaaacatctgagacttcacattccaataggcaaacaggttatccaatcggattaacttacgaaccagtttctcagtttcatcatgtaaacatggaacccagtattgatcagttgtctgcatgctcagattttgaagggaaataccaaatgacagcggtttgtcccgatttgtgatatcatcttcataacgaatatggatactggaaattttcacctgaagattttttatgatctgtgtaactaatttttctgcaaaagtgtcctgtttttccggcagatgttgttcttgatcaactactttttgttttgcttcttctattcttttcagttcctgttgctttgcttccatgagttgtttctcttcttttaaaggatcatattttattctagaagaaggcactataagtaaataaatttcttccaatacggcttcaacaggttgagtataaaggtttttccatggaattataagtttaagattacctatgtgaccaactttaactttaaatggtacatccagttgactcagggcattttctttaatttgaagattcttgagggccacagctcctttccagatgcccagagagagctgggacgtgtccaagtccaccacatagtcccccaagaaccggttcaacacgtccacgaccaccgactcgaaaaccatgttcctcagccgtggtgggcacggcagccggcccgtgcgctcctcctcccgccgccttccccacgcccctccctcgaggtaattcggttcaccggctccggggcggcttcagctgcggcgcccccgctggcccaacgcgcagccctagcgagcccagcgagagacggaggcggtcgctctcacgacgcgtgcgcaagtctgcgcgcggctggaggcggagcgcggcgcagacctgggcgcgcagccctgagagggaggaaaggcggctgcgcggccgcggctctggagggtgcccttttcgcgccgagcccggctcctctttcctgtcggccccgcctcctccccatcgcct

SEQ ID NO: 16704 - RNA, 3443 nt, Homo sapiens
  source 1..3443: mol_type = other RNA
taaagtgcttatagtgcaggtagtcaagagtgcttctctccaccagggttttgtagatggattcctcaaaaactcttttgaggtattgcctgggcttctcagtcgggttgatttcctcatcttctatttgatgggctaactgctctatggaaggaagatcttcctcctccttggaggctaagatttggcgtaactctttcctgagatcaataaaacgatcgtggaacagggccaggcaccacggctcggtgaagtagctatagagatctgtgatcaggttttcatcgtaccgagcacacaggttgttgaggagttgctcgtgctggccaaacaagcggatgtagttggaggcggggaagggctccctagaaaggcacgtgatggtttccaccattttatacttgttaatatgaattcggaagtaagtcccatttttcgcactgccggttactagttctaaaccataattaggctgtgccatttgtacctccaagggagttggaatggcaggcttggcaatatgcagataatggtaagacccaggaagaatgccccagagcactggagtctgaaaggcttggtgggtgtggtgaaggaggcgctgtagatggggtctgggtgcaggccgtcattccactgggccaggatcgcatcccggtacatagtgactccggcggctcctagcgcgtccgccacggcgctctccaccgagtagttgttgatgcaggtgatggtggaggcgggcgggggctgcacgaggtggatgcggctgccgctcacgccaaggtttaagagcgtctccacggtggtgtaagtatcaattgtattcccatagacaatgatattcccttctgtggtgatggagttattccttatccaaatcagtgccttaaagcaatcctcttcctcgttgagagtgaaatggttgcaaggaactttccccgtgtaccgccgctgactgctgttgggaacctccctgtttgtcaggtgttgactaatatcagcctctgtagggcatgggacctggtactgctgcccggtgcagaggatgaggtggtcgtagggcacgatctcgtccgtggaaagcacaacgtgcttggctgctcggtctatgccggtcattctacccaccacgacattaacccaggagcacagtgacatcagtgcataatctttatcattaaaacagtggtcgctggctaaaaatttcctttgttcagtgtccagaagtttttttcctgggagtccatgagttgaaatcagggtaagattattaaacttcatgtgagagcaaaataccaatgtctctaggaaggaaattccaacactggatgcaccaaccacaatgatcttggcattgacagtaattttaggttccaatgttagttttctgtttgtatggtttaaagcataactcatcggatccttggagaccgcctttgatggagcgtttatgccaagcttttccagaggatagacaatctgtcgtcgtggtcgcacgggaaccaagtaatgaagggcagatgtcagggagtgggcgtaggggttctggaactgaaagacagcaatcttgccttctctggattttgggtaaacacggtagtagagacaggatttaaagcctaaacgcaggatctccttcagaaagaacttggtgtagtgccggaaaatggggttgagggcaaagtgatgcatgtgcccgtgttcttcgcgctggtggtgactgaagtagatgaaatcttcaatgttgtaatgggaccgtatgtactcaatgtccatttcatttctgatcactgcaataccaactatttgttctgcaacttcagctacaaatgcctgcagcagtgttccatcagggtctttgcgagccttgttgtaacggtctaagtcctccaatatgcttttattcaacatgagggtgctgacaagattttccacaccaggagtatccaagagagtggcaaatcttatattaatggacttgagcaatccagcccggtggaagacgtagaggtcctgctcgagggtgcaggtgttgaaagggaccattttcacgaagttctggatgaggaagaactcgggggtgagatggggcagagaaattacacagaagttcttatcagaaaaaagactgaaaacaaaattcataaaatccagcgaccttgcttcatatttctcatcaatacaaaacagctgaatacaaaaagcagctgaggctcccctgtagatggggcggaagtggacgggctcttcaggcagtacgagcgatgccaagctcctactgctgacatggtgatactgtgcatatccagtggagatgtcactgagtttttctatgtcctccggttcactaacatttccactttggactgctgttaaagcttcctcggatgcagcttctctggcaatatttccctggatgttttccatggtatctggagagacaggttcctgcaactcctcgactattttttgggaaccttggctgctactcctgagctcagcatcttgacttcttcggacacttaggtcttgtggtgattccagaacgtcatcaggatgtgggaaacagagtccgtggaaagggcccaagtcaaagcactcatgcagcagttgcatgttcactcttgagcacacactcatgaacccaacagctgtgccttccacctcacacacaacagcatgattctcttcatcttgggcctctattagttcggccaggaagtattcaccgtaagtttccttcagaattgtgtcatagcgcataaatattggcatgagatcgtcatggtcttccaccctggctttgcgaacgtgcagctgaggatagtggctgtgcctgtgacatatatgcactgcaaagtcttcctcatacgtcagacacgggatgttccccacttggtcaaaaacagttatgagagttgagcctaggctcatgtaggatggcacgatgagaaatatgaagtgcagctctggcactgccttatacacggttcgaagaatctctttgcaacagccaacagaatactcatccacggccacaaagaggtgcatgaacaacgtattcaggggtgtgcatgggatgtcactgtcgagctcccggaacactgacacccagtcatcctgcttggcaacattccagttggggtagtccaggaaggtggcctgggccatgatctcctccttgtcattgcagagggtaacagcaaggttggccttttctagaagatagatgatatttagcttcccaaacagcttgcaggtaaattttctaataaggcttttgatacaataaacatcctgtgattctgttcttcggcaatgaacaacttctacctttcctcttggagaagtgagtactgacattttttatcctcatccgcagctccaggacgccgcactccacgcgctgccgcaaggaggacgcgcagcctggtcaccat

SEQ ID NO: 16705 - RNA, 3693 nt, Homo sapiens
  source 1..3693: mol_type = other RNA
taaagtgcttatagtgcaggtagtcaagagtgcttctctccaccagggttttgtagatggattcctcaaaaactcttttgaggtattgcctgggcttctcagtcgggttgatttcctcatcttctatttgatgggctaactgctctatggaaggaagatcttcctcctccttggaggctaagatttggcgtaactctttcctgagatcaataaaacgatcgtggaacagggccaggcaccacggctcggtgaagtagctatagagatctgtgatcaggttttcatcgtaccgagcacacaggttgttgaggagttgctcgtgctggccaaacaagcggatgtagttggaggcggggaagggctccctagaaaggcacgtgatggtttccaccattttatacttgttaatatgaattcggaagtaagtcccatttttcgcactgccggttactagttctaaaccataattaggctgtgccatttgtacctccaagggagttggaatggcaggcttggcaatatgcagataatggtaagacccaggaagaatgcccccttgaatcttggctcccttgtacatggggatgagccggtcaagattagctggtggctcggtcacaggctcaagggttggatcaaagagatgtagcatagctgctgccagctgaaagccaatttctttggaactgaagttgctgtgagtccactcatttgagtagtatctattggagaatttggtgagggagccagcagctctgatggctatgtcgttggtgtggaagttggtatcaatcacaagtcgactgtcatacacaagacatgcatcattgagggctttaaacgtttcataatccacattcttctcacagaagctgaagaacatagagcactggagtctgaaaggcttggtgggtgtggtgaaggaggcgctgtagatggggtctgggtgcaggccgtcattccactgggccaggatcgcatcccggtacatagtgactccggcggctcctagcgcgtccgccacggcgctctccaccgagtagttgttgatgcaggtgatggtggaggcgggcgggggctgcacgaggtggatgcggctgccgctcacgccaaggtttaagagcgtctccacggtggtgtaagtatcaattgtattcccatagacaatgatattcccttctgtggtgatggagttattccttatccaaatcagtgccttaaagcaatcctcttcctcgttgagagtgaaatggttgcaaggaactttccccgtgtaccgccgctgactgctgttgggaacctccctgtttgtcaggtgttgactaatatcagcctctgtagggcatgggacctggtactgctgcccggtgcagaggatgaggtggtcgtagggcacgatctcgtccgtggaaagcacaacgtgcttggctgctcggtctatgccggtcattctacccaccacgacattaacccaggagcacagtgacatcagtgcataatctttatcattaaaacagtggtcgctggctaaaaatttcctttgttcagtgtccagaagtttttttcctgggagtccatgagttgaaatcagggtaagattattaaacttcatgtgagagcaaaataccaatgtctctaggaaggaaattccaacactggatgcaccaaccacaatgatcttggcattgacagtaattttaggttccaatgttagttttctgtttgtatggtttaaagcataactcatcggatccttggagaccgcctttgatggagcgtttatgccaagcttttccagaggatagacaatctgtcgtcgtggtcgcacgggaaccaagtaatgaagggcagatgtcagggagtgggcgtaggggttctggaactgaaagacagcaatcttgccttctctggattttgggtaaacacggtagtagagacaggatttaaagcctaaacgcaggatctccttcagaaagaacttggtgtagtgccggaaaatggggttgagggcaaagtgatgcatgtgcccgtgttcttcgcgctggtggtgactgaagtagatgaaatcttcaatgttgtaatgggaccgtatgtactcaatgtcagggtctttgcgagccttgttgtaacggtctaagtcctccaatatgcttttattcaacatgagggtgctgacaagattttccacaccaggagtatccaagagagtggcaaatcttatattaatggacttgagcaatccagcccggtggaagacgtagaggtcctgctcgagggtgcaggtgttgaaagggaccattttcacgaagttctggatgaggaagaactcgggggtgagatggggcagagaaattacacagaagttcttatcagaaaaaagactgaaaacaaaattcataaaatccagcgaccttgcttcatatttctcatcaatacaaaacagctgaatacaaaaagcagctgaggctcccctgtagatggggcggaagtggacgggctcttcaggcagtacgagcgatgccaagctcctactgctgacatggtgatactgtgcatatccagtggagatgtcactgagtttttctatgtcctccggttcactaacatttccactttggactgctgttaaagcttcctcggatgcagcttctctggcaatatttccctggatgttttccatggtatctggagagacaggttcctgcaactcctcgactattttttgggaaccttggctgctactcctgagctcagcatcttgacttcttcggacacttaggtcttgtggtgattccagaacgtcatcaggatgtgggaaacagagtccgtggaaagggcccaagtcaaagcactcatgcagcagttgcatgttcactcttgagcacacactcatgaacccaacagctgtgccttccacctcacacacaacagcatgattctcttcatcttgggcctctattagttcggccaggaagtattcaccgtaagtttccttcagaattgtgtcatagcgcataaatattggcatgagatcgtcatggtcttccaccctggctttgcgaacgtgcagctgaggatagtggctgtgcctgtgacatatatgcactgcaaagtcttcctcatacgtcagacacgggatgttccccacttggtcaaaaacagttatgagagttgagcctaggctcatgtaggatggcacgatgagaaatatgaagtgcagctctggcactgccttatacacggttcgaagaatctctttgcaacagccaacagaatactcatccacggccacaaagaggtgcatgaacaacgtattcaggggtgtgcatgggatgtcactgtcgagctcccggaacactgacacccagtcatcctgcttggcaacattccagttggggtagtccaggaaggtggcctgggccatgatctcctccttgtcattgcagagggtaacagcaaggttggccttttctagaagatagatgatatttagcttcccaaacagcttgcaggtaaattttctaataaggcttttgatacaataaacatcctgtgattctgttcttcggcaatgaacaacttctacctttcctcttggagaagtgagtactgacattttttatcctcatccgcagctccaggacgccgcactccacgcgctgccgcaaggaggacgcgcagcctggtcaccat

SEQ ID NO: 16706 - RNA, 3523 nt, Homo sapiens
  source 1..3523: mol_type = other RNA
taaagtgcttatagtgcaggtagtcaagagtgcttctctccaccagggttttgtagatggattcctcaaaaactcttttgaggtattgcctgggcttctcagtcgggttgatttcctcatcttctatttgatgggctaactgctctatggaaggaagatcttcctcctccttggaggctaagatttggcgtaactctttcctgagatcaataaaacgatcgtggaacagggccaggcaccacggctcggtgaagtagctatagagatctgtgatcaggttttcatcgtaccgagcacacaggttgttgaggagttgctcgtgctggccaaacaagcggatgtagttggaggcggggaagggctccctagaaaggcacgtgatggtttccaccattttatacttgttaatatgaattcggaagtaagtcccatttttcgcactgccggttactagttctaaaccataattaggctgtgccatttgtacctccaagggagttggaatggcaggcttggcaatatgcagataatggtaagacccaggaagaatgcccccttgaatcttggctcccttgtacatggggatgagccggtcaagattagctggtggctcggtcacaggctcaagggttggatcaaagagatgtagcatagctgctgccagctgaaagccaatttctttggaactgaagttgctgtgagtccactcatttgagtagtatctattggagaatttggtgagggagccagcagctctgatggctatgtcgttggtgtggaagttggtatcaatcacaagtcgactgtcatacacaagacatgcatcattgagggctttaaacgtttcataatccacattcttctcacagaagctgaagaacatagagcactggagtctgaaaggcttggtgggtgtggtgaaggaggcgctgtagatggggtctgggtgcaggccgtcattccactgggccaggatcgcatcccggtacatagtgactccggcggctcctagcgcgtccgccacggcgctctccaccgagtagttgttgatgcaggtgatggtggaggcgggcgggggctgcacgaggtggatgcggctgccgctcacgccaaggtttaagagcgtctccacggtggtgtaagtatcaattgtattcccatagacaatgatattcccttctgtggtgatggagttattccttatccaaatcagtgccttaaagcaatcctcttcctcgttgagagtgaaatggttgcaaggaactttccccgtgtaccgccgctgactgctgttgggaacctccctgtttgtcaggtgttgactaatatcagcctctgtagggcatgggacctggtactgctgcccggtgcagaggatgaggtggtcgtagggcacgatctcgtccgtggaaagcacaacgtgcttggctgctcggtctatgccggtcattctacccaccacgacattaacccaggagcacagtgacatcagtgcataatctttatcattaaaacagtggtcgctggctaaaaatttcctttgttcagtgtccagaagtttttttcctgggagtccatgagttgaaatcagggtaagattattaaacttcatgtgagagcaaaataccaatgtctctaggaaggaaattccaacactggatgcaccaaccacaatgatcttggcattgacagtaattttaggttccaatgttagttttctgtttgtatggtttaaagcataactcatcggatccttggagaccgcctttgatggagcgtttatgccaagcttttccagaggatagacaatctgtcgtcgtggtcgcacgggaaccaagtaatgaagggcagatgtcagggagtgggcgtaggggttctggaactgaaagacagcaatcttgccttctctggattttgggtaaacacggtagtagagacaggatttaaagcctaaacgcaggatctccttcagaaagaacttggtgtagtgccggaaaatggggttgagggcaaagtgatgcatgtgcccgtgttcttcgcgctggtggtgactgaagtagatgaaatcttcaatgttgtaatgggaccgtatgtactcaatgtccatttcatttctgatcactgcaataccaactatttgttctgcaacttcagctacaaatgcctgcagcagtgttccatcagggtctttgcgagccttgttgtaacggtctaagtcctccaatatgcttttattcaacatgagggtgctgacaagattttccacaccaggagtatccaagagagtggcaaatcttatattaatggacttgagcaatccagcccggtggaagacgtagaggtcctgctcgagggtgcaggtgttgaaagggaccattttcacgaagttagaaaaaagactgaaaacaaaattcataaaatccagcgacctccggttcactaacatttccactttggactgctgttaaagcttcctcggatgcagcttctctggcaatatttccctggatgttttccatggtatctggagagacaggttcctgcaactcctcgactattttttgggaaccttggctgctactcctgagctcagcatcttgacttcttcggacacttaggtcttgtggtgattccagaacgtcatcaggatgtgggaaacagagtccgtggaaagggcccaagtcaaagcactcatgcagcagttgcatgttcactcttgagcacacactcatgaacccaacagctgtgccttccacctcacacacaacagcatgattctcttcatcttgggcctctattagttcggccaggaagtattcaccgtaagtttccttcagaattgtgtcatagcgcataaatattggcatgagatcgtcatggtcttccaccctggctttgcgaacgtgcagctgaggatagtggctgtgcctgtgacatatatgcactgcaaagtcttcctcatacgtcagacacgggatgttccccacttggtcaaaaacagttatgagagttgagcctaggctcatgtaggatggcacgatgagaaatatgaagtgcagctctggcactgccttatacacggttcgaagaatctctttgcaacagccaacagaatactcatccacggccacaaagaggtgcatgaacaacgtattcaggggtgtgcatgggatgtcactgtcgagctcccggaacactgacacccagtcatcctgcttggcaacattccagttggggtagtccaggaaggtggcctgggccatgatctcctccttgtcattgcagagggtaacagcaaggttggccttttctagaagatagatgatatttagcttcccaaacagcttgcaggtaaattttctaataaggcttttgatacaataaacatcctgtgattctgttcttcggcaatgaacaacttctacctttcctcttggagaagtgagtactgacattttttatcctcatccgcagctccaggacgccgcactccacgcgctgccgcaaggaggacgcgcagcct

SEQ ID NO: 16707 - RNA, 3711 nt, Homo sapiens
  source 1..3711: mol_type = other RNA
taaagtgcttatagtgcaggtagtcaagagtgcttctctccaccagggttttgtagatggattcctcaaaaactcttttgaggtattgcctgggcttctcagtcgggttgatttcctcatcttctatttgatgggctaactgctctatggaaggaagatcttcctcctccttggaggctaagatttggcgtaactctttcctgagatcaataaaacgatcgtggaacagggccaggcaccacggctcggtgaagtagctatagagatctgtgatcaggttttcatcgtaccgagcacacaggttgttgaggagttgctcgtgctggccaaacaagcggatgtagttggaggcggggaagggctccctagaaaggcacgtgatggtttccaccattttatacttgttaatatgaattcggaagtaagtcccatttttcgcactgccggttactagttctaaaccataattaggctgtgccatttgtacctccaagggagttggaatggcaggcttggcaatatgcagataatggtaagacccaggaagaatgcccccttgaatcttggctcccttgtacatggggatgagccggtcaagattagctggtggctcggtcacaggctcaagggttggatcaaagagatgtagcatagctgctgccagctgaaagccaatttctttggaactgaagttgctgtgagtccactcatttgagtagtatctattggagaatttggtgagggagccagcagctctgatggctatgtcgttggtgtggaagttggtatcaatcacaagtcgactgtcatacacaagacatgcatcattgagggctttaaacgtttcataatccacattcttctcacagaagctgaagaacatagagcactggagtctgaaaggcttggtgggtgtggtgaaggaggcgctgtagatggggtctgggtgcaggccgtcattccactgggccaggatcgcatcccggtacatagtgactccggcggctcctagcgcgtccgccacggcgctctccaccgagtagttgttgatgcaggtgatggtggaggcgggcgggggctgcacgaggtggatgcggctgccgctcacgccaaggtttaagagcgtctccacggtggtgtaagtatcaattgtattcccatagacaatgatattcccttctgtggtgatggagttattccttatccaaatcagtgccttaaagcaatcctcttcctcgttgagagtgaaatggttgcaaggaactttccccgtgtaccgccgctgactgctgttgggaacctccctgtttgtcaggtgttgactaatatcagcctctgtagggcatgggacctggtactgctgcccggtgcagaggatgaggtggtcgtagggcacgatctcgtccgtggaaagcacaacgtgcttggctgctcggtctatgccggtcattctacccaccacgacattaacccaggagcacagtgacatcagtgcataatctttatcattaaaacagtggtcgctggctaaaaatttcctttgttcagtgtccagaagtttttttcctgggagtccatgagttgaaatcagggtaagattattaaacttcatgtgagagcaaaataccaatgtctctaggaaggaaattccaacactggatgcaccaaccacaatgatcttggcattgacagtaattttaggttccaatgttagttttctgtttgtatggtttaaagcataactcatcggatccttggagaccgcctttgatggagcgtttatgccaagcttttccagaggatagacaatctgtcgtcgtggtcgcacgggaaccaagtaatgaagggcagatgtcagggagtgggcgtaggggttctggaactgaaagacagcaatcttgccttctctggattttgggtaaacacggtagtagagacaggatttaaagcctaaacgcaggatctccttcagaaagaacttggtgtagtgccggaaaatggggttgagggcaaagtgatgcatgtgcccgtgttcttcgcgctggtggtgactgaagtagatgaaatcttcaatgttgtaatgggaccgtatgtactcaatgtccatttcatttctgatcactgcaataccaactatttgttctgcaacttcagctacaaatgcctgcagcagtgttccatcagggtctttgcgagccttgttgtaacggtctaagtcctccaatatgcttttattcaacatgagggtgctgacaagattttccacaccaggagtatccaagagagtggcaaatcttatattaatggacttgagcaatccagcccggtggaagacgtagaggtcctgctcgagggtgcaggtgttgaaagggaccattttcacgaagttagaaaaaagactgaaaacaaaattcataaaatccagcgaccttgcttcatatttctcatcaatacaaaacagctgaatacaaaaagcagctgaggctcccctgtagatggggcggaagtggacgggctcttcaggcagtacgagcgatgccaagctcctactgctgacatggtgatactgtgcatatccagtggagatgtcactgagtttttctatgtcctccggttcactaacatttccactttggactgctgttaaagcttcctcggatgcagcttctctggcaatatttccctggatgttttccatggtatctggagagacaggttcctgcaactcctcgactattttttgggaaccttggctgctactcctgagctcagcatcttgacttcttcggacacttaggtcttgtggtgattccagaacgtcatcaggatgtgggaaacagagtccgtggaaagggcccaagtcaaagcactcatgcagcagttgcatgttcactcttgagcacacactcatgaacccaacagctgtgccttccacctcacacacaacagcatgattctcttcatcttgggcctctattagttcggccaggaagtattcaccgtaagtttccttcagaattgtgtcatagcgcataaatattggcatgagatcgtcatggtcttccaccctggctttgcgaacgtgcagctgaggatagtggctgtgcctgtgacatatatgcactgcaaagtcttcctcatacgtcagacacgggatgttccccacttggtcaaaaacagttatgagagttgagcctaggctcatgtaggatggcacgatgagaaatatgaagtgcagctctggcactgccttatacacggttcgaagaatctctttgcaacagccaacagaatactcatccacggccacaaagaggtgcatgaacaacgtattcaggggtgtgcatgggatgtcactgtcgagctcccggaacactgacacccagtcatcctgcttggcaacattccagttggggtagtccaggaaggtggcctgggccatgatctcctccttgtcattgcagagggtaacagcaaggttggccttttctagaagatagatgatatttagcttcccaaacagcttgcaggtaaattttctaataaggcttttgatacaataaacatcctgtgattctgttcttcggcaatgaacaacttctacctttcctcttggagaagtgagtactgacattttttatcctcatccgcagctccaggacgccgcactccacgcgctgccgcaaggaggacgcgcagcctggtcaccat

SEQ ID NO: 16708 - RNA, 3583 nt, Homo sapiens
  source 1..3583: mol_type = other RNA
taaagtgcttatagtgcaggtagtcaagagtgcttctctccaccagggttttgtagatggattcctcaaaaactcttttgaggtattgcctgggcttctcagtcgggttgatttcctcatcttctatttgatgggctaactgctctatggaaggaagatcttcctcctccttggaggctaagatttggcgtaactctttcctgagatcaataaaacgatcgtggaacagggccaggcaccacggctcggtgaagtagctatagagatctgtgatcaggttttcatcgtaccgagcacacaggttgttgaggagttgctcgtgctggccaaacaagcggatgtagttggaggcggggaagggctccctagaaaggcacgtgatggtttccaccattttatacttgttaatatgaattcggaagtaagtcccatttttcgcactgccggttactagttctaaaccataattaggctgtgccatttgtacctccaagggagttggaatggcaggcttggcaatatgcagataatggtaagacccaggaagaatgcccccttgaatcttggctcccttgtacatggggatgagccggtcaagattagctggtggctcggtcacaggctcaagggttggatcaaagagatgtagcatagctgctgccagctgaaagccaatttctttggaactgaagttgctgtgagtccactcatttgagtagtatctattggagaatttggtgagggagccagcagctctgatggctatgtcgttggtgtggaagttggtatcaatcacaagtcgactgtcatacacaagacatgcatcattgagggctttaaacgtttcataatccacattcttctcacagaagctgaagaacatagagcactggagtctgaaaggcttggtgggtgtggtgaaggaggcgctgtagatggggtctgggtgcaggccgtcattccactgggccaggatcgcatcccggtacatagtgactccggcggctcctagcgcgtccgccacggcgctctccaccgagtagttgttgatgcaggtgatggtggaggcgggcgggggctgcacgaggtggatgcggctgccgctcacgccaaggtttaagagcgtctccacggtggtgtaagtatcaattgtattcccatagacaatgatattcccttctgtggtgatggagttattccttatccaaatcagtgccttaaagcaatcctcttcctcgttgagagtgaaatggttgcaaggaactttccccgtgtaccgccgctgactgctgttgggaacctccctgtttgtcaggtgttgactaatatcagcctctgtagggcatgggacctggtactgctgcccggtgcagaggatgaggtggtcgtagggcacgatctcgtccgtggaaagcacaacgtgcttggctgctcggtctatgccggtcattctacccaccacgacattaacccaggagcacagtgacatcagtgcataatctttatcattaaaacagtggtcgctggctaaaaatttcctttgttcagtgtccagaagtttttttcctgggagtccatgagttgaaatcagggtaagattattaaacttcatgtgagagcaaaataccaatgtctctaggaaggaaattccaacactggatgcaccaaccacaatgatcttggcattgacagtaattttaggttccaatgttagttttctgtttgtatggtttaaagcataactcatcggatccttggagaccgcctttgatggagcgtttatgccaagcttttccagaggatagacaatctgtcgtcgtggtcgcacgggaaccaagtaatgaagggcagatgtcagggagtgggcgtaggggttctggaactgaaagacagcaatcttgccttctctggattttgggtaaacacggtagtagagacaggatttaaagcctaaacgcaggatctccttcagaaagaacttggtgtagtgccggaaaatggggttgagggcaaagtgatgcatgtgcccgtgttcttcgcgctggtggtgactgaagtagatgaaatcttcaatgttgtaatgggaccgtatgtactcaatgtccatttcatttctgatcactgcaataccaactatttgttctgcaacttcagctacaaatgcctgcagcagtgttccatcagggtctttgcgagccttgttgtaacggtctaagtcctccaatatgcttttattcaacatgagggtgctgacaagattttccacaccaggagtatccaagagagtggcaaatcttatattaatggacttgagcaatccagcccggtggaagacgtagaggtcctgctcgagggtgcaggtgttgaaagggaccattttcacgaagttctggatgaggaagaactcgggggtgagatggggcagagaaattacacagaagttcttatcagaaaaaagactgaaaacaaaattcataaaatccagcgacctccggttcactaacatttccactttggactgctgttaaagcttcctcggatgcagcttctctggcaatatttccctggatgttttccatggtatctggagagacaggttcctgcaactcctcgactattttttgggaaccttggctgctactcctgagctcagcatcttgacttcttcggacacttaggtcttgtggtgattccagaacgtcatcaggatgtgggaaacagagtccgtggaaagggcccaagtcaaagcactcatgcagcagttgcatgttcactcttgagcacacactcatgaacccaacagctgtgccttccacctcacacacaacagcatgattctcttcatcttgggcctctattagttcggccaggaagtattcaccgtaagtttccttcagaattgtgtcatagcgcataaatattggcatgagatcgtcatggtcttccaccctggctttgcgaacgtgcagctgaggatagtggctgtgcctgtgacatatatgcactgcaaagtcttcctcatacgtcagacacgggatgttccccacttggtcaaaaacagttatgagagttgagcctaggctcatgtaggatggcacgatgagaaatatgaagtgcagctctggcactgccttatacacggttcgaagaatctctttgcaacagccaacagaatactcatccacggccacaaagaggtgcatgaacaacgtattcaggggtgtgcatgggatgtcactgtcgagctcccggaacactgacacccagtcatcctgcttggcaacattccagttggggtagtccaggaaggtggcctgggccatgatctcctccttgtcattgcagagggtaacagcaaggttggccttttctagaagatagatgatatttagcttcccaaacagcttgcaggtaaattttctaataaggcttttgatacaataaacatcctgtgattctgttcttcggcaatgaacaacttctacctttcctcttggagaagtgagtactgacattttttatcctcatccgcagctccaggacgccgcactccacgcgctgccgcaaggaggacgcgcagcct

SEQ ID NO: 16709 - RNA, 2553 nt, Homo sapiens
  source 1..2553: mol_type = other RNA
taaagtgcttatagtgcaggtagtcaagagtgcttctctccaccagggttttgtagatggattcctcaaaaactcttttgaggtattgcctgggcttctcagtcgggttgatttcctcatcttctatttgatgggctaactgctctatggaaggaagatcttcctcctccttggaggctaagatttggcgtaactctttcctgagatcaataaaacgatcgtggaacagggccaggcaccacggctcggtgaagtagctatagagatctgtgatcaggttttcatcgtaccgagcacacaggttgttgaggagttgctcgtgctggccaaacaagcggatgtagttggaggcggggaagggctccctagaaaggcacgtgatggtttccaccattttatacttgttaatatgaattcggaagtaagtcccatttttcgcactgccggttactagttctaaaccataattaggctgtgccatttgtacctccaagggagttggaatggcaggcttggcaatatgcagataatggtaagacccaggaagaatgcccccttgaatcttggctcccttgtacatggggatgagccggtcaagattagctggtggctcggtcacaggctcaagggttggatcaaagagatgtagcatagctgctgccagctgaaagccaatttctttggaactgaagttgctgtgagtccactcatttgagtagtatctattggagaatttggtgagggagccagcagctctgatggctatgtcgttggtgtggaagttggtatcaatcacaagtcgactgtcatacacaagacatgcatcattgagggctttaaacgtttcataatccacattcttctcacagaagctgaagaacatagagcactggagtctgaaaggcttggtgggtgtggtgaaggaggcgctgtagatggggtctgggtgcaggccgtcattccactgggccaggatcgcatcccggtacatagtgactccggcggctcctagcgcgtccgccacggcgctctccaccgagtagttgttgatgcaggtgatggtggaggcgggcgggggctgcacgaggtggatgcggctgccgctcacgccaaggtttaagagcgtctccacggtggtgtaagtatcaattgtattcccatagacaatgatattcccttctgtggtgatggagttattccttatccaaatcagtgccttaaagcaatcctcttcctcgttgagagtgaaatggttgcaaggaactttccccgtgtaccgccgctgactgctgttgggaacctccctgtttgtcaggtgttgactaatatcagcctctgtagggcatgggacctggtactgctgcccggtgcagaggatgaggtggtcgtagggcacgatctcgtccgtggaaagcacaacgtgcttggctgctcggtctatgccggtcattctacccaccacgacattaacccaggagcacagtgacatcagtgcataatctttatcattaaaacagtggtcgctggctaaaaatttcctttgttcagtgtccagaagtttttttcctgggagtccatgagttgaaatcagggtaagattattaaacttcatgtgagagcaaaataccaatgtctctaggaaggaaattccaacactggatgcaccaaccacaatgatcttggcattgacagtaattttaggttccaatgttagttttctgtttgtatggtttaaagcataactcatcggatccttggagaccgcctttgatggagcgtttatgccaagcttttccagaggatagacaatctgtcgtcgtggtcgcacgggaaccaagtaatgaagggcagatgtcagggagtgggcgtaggggttctggaactgaaagacagcaatcttgccttctctggattttgggtaaacacggtagtagagacaggatttaaagcctaaacgcaggatctccttcagaaagaacttggtgtagtgccggaaaatggggttgagggcaaagtgatgcatgtgcccgtgttcttcgcgctggtggtgactgaagtagatgaaatcttcaatgttgtaatgggaccgtatgtactcaatgtccatttcatttctgatcactgcaataccaactatttgttctgcaacttcagctacaaatgcctgcagcagtgttccatcagggtctttgcgagccttgttgtaacggtctaagtcctccaatatgcttttattcaacatgagggtgctgacaagattttccacaccaggagtatccaagagagtggcaaatcttatattaatggacttgagcaatccagcccggtggaagacgtagaggtcctgctcgagggtgcaggtgttgaaagggaccattttcacgaagttctggatgaggaagaactcgggggtgagatggggcagagaaattacacagaagttcttatcagaaaaaagactgaaaacaaaattcataaaatccagcgacctggatgttttccatggtatctggagagacaggttcctgcaactcctcgactattttttgggaa

SEQ ID NO: 16710 - RNA, 4082 nt, Homo sapiens
  source 1..4082: mol_type = other RNA
taaagtgcttatagtgcaggtagtcaagagtgcttctctccaccagggttttgtagatggattcctcaaaaactcttttgaggtattgcctgggcttctcagtcgggttgatttcctcatcttctatttgatgggctaactgctctatggaaggaagatcttcctcctccttggaggctaagatttggcgtaactctttcctgagatcaataaaacgatcgtggaacagggccaggcaccacggctcggtgaagtagctatagagatctgtgatcaggttttcatcgtaccgagcacacaggttgttgaggagttgctcgtgctggccaaacaagcggatgtagttggaggcggggaagggctccctagaaaggcacgtgatggtttccaccattttatacttgttaatatgaattcggaagtaagtcccatttttcgcactgccggttactagttctaaaccataattaggctgtgccatttgtacctccaagggagttggaatggcaggcttggcaatatgcagataatggtaagacccaggaagaatgcccccttgaatcttggctcccttgtacatggggatgagccggtcaagattagctggtggctcggtcacaggctcaagggttggatcaaagagatgtagcatagctgctgccagctgaaagccaatttctttggaactgaagttgctgtgagtccactcatttgagtagtatctattggagaatttggtgagggagccagcagctctgatggctatgtcgttggtgtggaagttggtatcaatcacaagtcgactgtcatacacaagacatgcatcattgagggctttaaacgtttcataatccacattcttctcacagaagctgaagaacatagagcactggagtctgaaaggcttggtgggtgtggtgaaggaggcgctgtagatggggtctgggtgcaggccgtcattccactgggccaggatcgcatcccggtacatagtgactccggcggctcctagcgcgtccgccacggcgctctccaccgagtagttgttgatgcaggtgatggtggaggcgggcgggggctgcacgaggtggatgcggctgccgctcacgccaaggtttaagagcgtctccacggtggtgtaagtatcaattgtattcccatagacaatgatattcccttctgtggtgatggagttattccttatccaaatcagtgccttaaagcaatcctcttcctcgttgagagtgaaatggttgcaaggaactttccccgtgtaccgccgctgactgctgttgggaacctccctgtttgtcaggtgttgactaatatcagcctctgtagggcatgggacctggtactgctgcccggtgcagaggatgaggtggtcgtagggcacgatctcgtccgtggaaagcacaacgtgcttggctgctcggtctatgccggtcattctacccaccacgacattaacccaggagcacagtgacatcagtgcataatctttatcattaaaacagtggtcgctggctaaaaatttcctttgttcagtgtccagaagtttttttcctgggagtccatgagttgaaatcagggtaagattattaaacttcatgtgagagcaaaataccaatgtctctaggaaggaaattccaacactggatgcaccaaccacaatgatcttggcattgacagtaattttaggttccaatgttagttttctgtttgtatggtttaaagcataactcatcggatccttggagaccgcctttgatggagcgtttatgccaagcttttccagaggatagacaatctgtcgtcgtggtcgcacgggaaccaagtaatgaagggcagatgtcagggagtgggcgtaggggttctggaactgaaagacagcaatcttgccttctctggattttgggtaaacacggtagtagagacaggatttaaagcctaaacgcaggatctccttcagaaagaacttggtgtagtgccggaaaatggggttgagggcaaagtgatgcatgtgcccgtgttcttcgcgctggtggtgactgaagtagatgaaatcttcaatgttgtaatgggaccgtatgtactcaatgtccatttcatttctgatcactgcaataccaactatttgttctgcaacttcagctacaaatgcctgcagcagtgttccatcagggtctttgcgagccttgttgtaacggtctaagtcctccaatatgcttttattcaacatgagggtgctgacaagattttccacaccaggagtatccaagagagtggcaaatcttatattaatggacttgagcaatccagcccggtggaagacgtagaggtcctgctcgagggtgcaggtgttgaaagggaccattttcacgaagttctggatgaggaagaactcgggggtgagatggggcagagaaattacacagaagttcttatcagaaaaaagactgaaaacaaaattcataaaatccagcgaccttgcttcatatttctcatcaatacaaaacagctgaatacaaaaagcagctgaggctcccctgtagatggggcggaagtggacgggctcttcaggcagtacgagcgatgccaagctcctactgctgacatggtgatactgtgcatatccagtggagatgtcactgagtttttctatgtcctccggttcactaacatttccactttggactgctgttaaagcttcctcggatgcagcttctctggcaatatttccctggatgttttccatggtatctggagagacaggttcctgcaactcctcgactattttttgggaaccttggctgctactcctgagctcagcatcttgacttcttcggacacttaggtcttgtggtgattccagaacgtcatcaggatgtgggaaacagagtccgtggaaagggcccaagtcaaagcactcatgcagcagttgcatgttcactcttgagcacacactcatgaacccaacagctgtgccttccacctcacacacaacagcatgattctcttcatcttgggcctctattagttcggccaggaagtattcaccgtaagtttccttcagaattgtgtcatagcgcataaatattggcatgagatcgtcatggtcttccaccctcaacacgaattcttctgggaaaaatagaaaaacatccaaatcttggagttctgaagaggctctctcttaagccctttcccaaaatggataaagaggaacttgttctgctaaatgcattccttggggtaattgataatttatgatcttgcatcagcccgagtgctaatgataaagtatgacatcagcctcacatagtctcaaatggcatatgacaaagtccagccccacagaaacaaaacaccccagctatggaaaacaactcatgcagtcaaatgtttcaacgtgactgttctgaggcaatgagcgctgcctgtcaaagtcaggatgcaaggagagccactgtgaatttggcaccgcagcgtcacatgccctggcactgacaggccgcacagtgttccagtggcgatgaagatgcggagtttatagatcagcacagagtgcaacggaaatagtacaattctctgagcgaaaagcaaagttactttatatcttccattctgaatgtgtcttggagggggcagcaatgtgcttgttaacgtcatcaattatacaatattttattttaacttccctggaggaaacaaaaggtccacctcataaacacttatcaatctctcagacacccagatttccatcagactctgaaaactgtgccatgtgaaatggagttgaacacacaccttaaggaaatcaaccccctttcaggacaccctacttgggaaatgggtgtcttctaagtccacagctagaaatgagccggtagctctcactggcttcctggaaggtggggagaagtgaggacaaactccctcagcacttccaccagtcggttagctgagcttgctaggagcaccgcgacatccagaacatgcagaactctccctcgcagcctgatgggtctctgggtgacacgcagatcctgacattgcttcatcacctccacagcctggct

SEQ ID NO: 16711 - RNA, 3771 nt, Homo sapiens
  source 1..3771: mol_type = other RNA
taaagtgcttatagtgcaggtagtcaagagtgcttctctccaccagggttttgtagatggattcctcaaaaactcttttgaggtattgcctgggcttctcagtcgggttgatttcctcatcttctatttgatgggctaactgctctatggaaggaagatcttcctcctccttggaggctaagatttggcgtaactctttcctgagatcaataaaacgatcgtggaacagggccaggcaccacggctcggtgaagtagctatagagatctgtgatcaggttttcatcgtaccgagcacacaggttgttgaggagttgctcgtgctggccaaacaagcggatgtagttggaggcggggaagggctccctagaaaggcacgtgatggtttccaccattttatacttgttaatatgaattcggaagtaagtcccatttttcgcactgccggttactagttctaaaccataattaggctgtgccatttgtacctccaagggagttggaatggcaggcttggcaatatgcagataatggtaagacccaggaagaatgcccccttgaatcttggctcccttgtacatggggatgagccggtcaagattagctggtggctcggtcacaggctcaagggttggatcaaagagatgtagcatagctgctgccagctgaaagccaatttctttggaactgaagttgctgtgagtccactcatttgagtagtatctattggagaatttggtgagggagccagcagctctgatggctatgtcgttggtgtggaagttggtatcaatcacaagtcgactgtcatacacaagacatgcatcattgagggctttaaacgtttcataatccacattcttctcacagaagctgaagaacatagagcactggagtctgaaaggcttggtgggtgtggtgaaggaggcgctgtagatggggtctgggtgcaggccgtcattccactgggccaggatcgcatcccggtacatagtgactccggcggctcctagcgcgtccgccacggcgctctccaccgagtagttgttgatgcaggtgatggtggaggcgggcgggggctgcacgaggtggatgcggctgccgctcacgccaaggtttaagagcgtctccacggtggtgtaagtatcaattgtattcccatagacaatgatattcccttctgtggtgatggagttattccttatccaaatcagtgccttaaagcaatcctcttcctcgttgagagtgaaatggttgcaaggaactttccccgtgtaccgccgctgactgctgttgggaacctccctgtttgtcaggtgttgactaatatcagcctctgtagggcatgggacctggtactgctgcccggtgcagaggatgaggtggtcgtagggcacgatctcgtccgtggaaagcacaacgtgcttggctgctcggtctatgccggtcattctacccaccacgacattaacccaggagcacagtgacatcagtgcataatctttatcattaaaacagtggtcgctggctaaaaatttcctttgttcagtgtccagaagtttttttcctgggagtccatgagttgaaatcagggtaagattattaaacttcatgtgagagcaaaataccaatgtctctaggaaggaaattccaacactggatgcaccaaccacaatgatcttggcattgacagtaattttaggttccaatgttagttttctgtttgtatggtttaaagcataactcatcggatccttggagaccgcctttgatggagcgtttatgccaagcttttccagaggatagacaatctgtcgtcgtggtcgcacgggaaccaagtaatgaagggcagatgtcagggagtgggcgtaggggttctggaactgaaagacagcaatcttgccttctctggattttgggtaaacacggtagtagagacaggatttaaagcctaaacgcaggatctccttcagaaagaacttggtgtagtgccggaaaatggggttgagggcaaagtgatgcatgtgcccgtgttcttcgcgctggtggtgactgaagtagatgaaatcttcaatgttgtaatgggaccgtatgtactcaatgtccatttcatttctgatcactgcaataccaactatttgttctgcaacttcagctacaaatgcctgcagcagtgttccatcagggtctttgcgagccttgttgtaacggtctaagtcctccaatatgcttttattcaacatgagggtgctgacaagattttccacaccaggagtatccaagagagtggcaaatcttatattaatggacttgagcaatccagcccggtggaagacgtagaggtcctgctcgagggtgcaggtgttgaaagggaccattttcacgaagttctggatgaggaagaactcgggggtgagatggggcagagaaattacacagaagttcttatcagaaaaaagactgaaaacaaaattcataaaatccagcgaccttgcttcatatttctcatcaatacaaaacagctgaatacaaaaagcagctgaggctcccctgtagatggggcggaagtggacgggctcttcaggcagtacgagcgatgccaagctcctactgctgacatggtgatactgtgcatatccagtggagatgtcactgagtttttctatgtcctccggttcactaacatttccactttggactgctgttaaagcttcctcggatgcagcttctctggcaatatttccctggatgttttccatggtatctggagagacaggttcctgcaactcctcgactattttttgggaaccttggctgctactcctgagctcagcatcttgacttcttcggacacttaggtcttgtggtgattccagaacgtcatcaggatgtgggaaacagagtccgtggaaagggcccaagtcaaagcactcatgcagcagttgcatgttcactcttgagcacacactcatgaacccaacagctgtgccttccacctcacacacaacagcatgattctcttcatcttgggcctctattagttcggccaggaagtattcaccgtaagtttccttcagaattgtgtcatagcgcataaatattggcatgagatcgtcatggtcttccaccctggctttgcgaacgtgcagctgaggatagtggctgtgcctgtgacatatatgcactgcaaagtcttcctcatacgtcagacacgggatgttccccacttggtcaaaaacagttatgagagttgagcctaggctcatgtaggatggcacgatgagaaatatgaagtgcagctctggcactgccttatacacggttcgaagaatctctttgcaacagccaacagaatactcatccacggccacaaagaggtgcatgaacaacgtattcaggggtgtgcatgggatgtcactgtcgagctcccggaacactgacacccagtcatcctgcttggcaacattccagttggggtagtccaggaaggtggcctgggccatgatctcctccttgtcattgcagagggtaacagcaaggttggccttttctagaagatagatgatatttagcttcccaaacagcttgcaggtaaattttctaataaggcttttgatacaataaacatcctgtgattctgttcttcggcaatgaacaacttctacctttcctcttggagaagtgagtactgacattttttatcctcatccgcagctccaggacgccgcactccacgcgctgccgcaaggaggacgcgcagcctggtcaccat

SEQ ID NO: 16712 - RNA, 3806 nt, Homo sapiens
  source 1..3806: mol_type = other RNA
taaagtgcttatagtgcaggtagtcaagagtgcttctctccaccagggttttgtagatggattcctcaaaaactcttttgaggtattgcctgggcttctcagtcgggttgatttcctcatcttctatttgatgggctaactgctctatggaaggaagatcttcctcctccttggaggctaagatttggcgtaactctttcctgagatcaataaaacgatcgtggaacagggccaggcaccacggctcggtgaagtagctatagagatctgtgatcaggttttcatcgtaccgagcacacaggttgttgaggagttgctcgtgctggccaaacaagcggatgtagttggaggcggggaagggctccctagaaaggcacgtgatggtttccaccattttatacttgttaatatgaattcggaagtaagtcccatttttcgcactgccggttactagttctaaaccataattaggctgtgccatttgtacctccaagggagttggaatggcaggcttggcaatatgcagataatggtaagacccaggaagaatgcccccttgaatcttggctcccttgtacatggggatgagccggtcaagattagctggtggctcggtcacaggctcaagggttggatcaaagagatgtagcatagctgctgccagctgaaagccaatttctttggaactgaagttgctgtgagtccactcatttgagtagtatctattggagaatttggtgagggagccagcagctctgatggctatgtcgttggtgtggaagttggtatcaatcacaagtcgactgtcatacacaagacatgcatcattgagggctttaaacgtttcataatccacattcttctcacagaagctgaagaacatagagcactggagtctgaaaggcttggtgggtgtggtgaaggaggcgctgtagatggggtctgggtgcaggccgtcattccactgggccaggatcgcatcccggtacatagtgactccggcggctcctagcgcgtccgccacggcgctctccaccgagtagttgttgatgcaggtgatggtggaggcgggcgggggctgcacgaggtggatgcggctgccgctcacgccaaggtttaagagcgtctccacggtggtgtaagtatcaattgtattcccatagacaatgatattcccttctgtggtgatggagttattccttatccaaatcagtgccttaaagcaatcctcttcctcgttgagagtgaaatggttgcaaggaactttccccgtgtaccgccgctgactgctgttgggaacctccctgtttgtcaggtgttgactaatatcagcctctgtagggcatgggacctggtactgctgcccggtgcagaggatgaggtggtcgtagggcacgatctcgtccgtggaaagcacaacgtgcttggctgctcggtctatgccggtcattctacccaccacgacattaacccaggagcacagtgacatcagtgcataatctttatcattaaaacagtggtcgctggctaaaaatttcctttgttcagtgtccagaagtttttttcctgggagtccatgagttgaaatcagggtaagattattaaacttcatgtgagagcaaaataccaatgtctctaggaaggaaattccaacactggatgcaccaaccacaatgatcttggcattgacagtaattttaggttccaatgttagttttctgtttgtatggtttaaagcataactcatcggatccttggagaccgcctttgatggagcgtttatgccaagcttttccagaggatagacaatctgtcgtcgtggtcgcacgggaaccaagtaatgaagggcagatgtcagggagtgggcgtaggggttctggaactgaaagacagcaatcttgccttctctggattttgggtaaacacggtagtagagacaggatttaaagcctaaacgcaggatctccttcagaaagaacttggtgtagtgccggaaaatggggttgagggcaaagtgatgcatgtgcccgtgttcttcgcgctggtggtgactgaagtagatgaaatcttcaatgttgtaatgggaccgtatgtactcaatgtccatttcatttctgatcactgcaataccaactatttgttctgcaacttcagctacaaatgcctgcagcagtgttccatcagggtctttgcgagccttgttgtaacggtctaagtcctccaatatgcttttattcaacatgagggtgctgacaagattttccacaccaggagtatccaagagagtggcaaatcttatattaatggacttgagcaatccagcccggtggaagacgtagaggtcctgctcgagggtgcaggtgttgaaagggaccattttcacgaagttctggatgaggaagaactcgggggtgagatggggcagagaaattacacagaagttcttatcagaaaaaagactgaaaacaaaattcataaaatccagcgaccttgcttcatatttctcatcaatacaaaacagctgaatacaaaaagcagctgaggctcccctgtagatggggcggaagtggacgggctcttcaggcagtacgagcgatgccaagctcctactgctgacatggtgatactgtgcatatccagtggagatgtcactgagtttttctatgtcctccggttcactaacatttccactttggactgctgttaaagcttcctcggatgcagcttctctggcaatatttccctggatgttttccatggtatctggagagacaggttcctgcaactcctcgactattttttgggaaccttggctgctactcctgagctcagcatcttgacttcttcggacacttaggtcttgtggtgattccagaacgtcatcaggatgtgggaaacagagtccgtggaaagggcccaagtcaaagcactcatgcagcagttgcatgttcactcttgagcacacactcatgaacccaacagctgtgccttccacctcacacacaacagcatgattctcttcatcttgggcctctattagttcggccaggaagtattcaccgtaagtttccttcagaattgtgtcatagcgcataaatattggcatgagatcgtcatggtcttccaccctggctttgcgaacgtgcagctgaggatagtggctgtgcctgtgacatatatgcactgcaaagtcttcctcatacgtcagacacgggatgttccccacttggtcaaaaacagttatgagagttgagcctaggctcatgtaggatggcacgatgagaaatatgaagtgcagctctggcactgccttatacacggttcgaagaatctctttgcaacagccaacagaatactcatccacggccacaaagaggtgcatgaacaacgtattcaggggtgtgcatgggatgtcactgtcgagctcccggaacactgacacccagtcatcctgcttggcaacattccagttggggtagtccaggaaggtggcctgggccatgatctcctccttgtcattgcagagggtaacagcaaggttggccttttctagaagatagatgatatttagcttcccaaacagcttgcaggtaaattttctaataaggcttttgatacaataaacatcctgtgattctgttcttcggcaatgaacaacttctacctttcctcttggagaagtgagtactgacattttttatcctggggatgcgccctggacgccctgcaccgcagtccttgcgtcgctgctagtcagcacggcgttacccacctcatccgcagctccaggacgccgcactccacgc

SEQ ID NO: 16713 - RNA, 3629 nt, Homo sapiens
  source 1..3629: mol_type = other RNA
taaagtgcttatagtgcaggtagtcaagagtgcttctctccaccagggttttgtagatggattcctcaaaaactcttttgaggtattgcctgggcttctcagtcgggttgatttcctcatcttctatttgatgggctaactgctctatggaaggaagatcttcctcctccttggaggctaagatttggcgtaactctttcctgagatcaataaaacgatcgtggaacagggccaggcaccacggctcggtgaagtagctatagagatctgtgatcaggttttcatcgtaccgagcacacaggttgttgaggagttgctcgtgctggccaaacaagcggatgtagttggaggcggggaagggctccctagaaaggcacgtgatggtttccaccattttatacttgttaatatgaattcggaagtaagtcccatttttcgcactgccggttactagttctaaaccataattaggctgtgccatttgtacctccaagggagttggaatggcaggcttggcaatatgcagataatggtaagacccaggaagaatgcccccttgaatcttggctcccttgtacatggggatgagccggtcaagattagctggtggctcggtcacaggctcaagggttggatcaaagagatgtagcatagctgctgccagctgaaagccaatttctttggaactgaagttgctgtgagtccactcatttgagtagtatctattggagaatttggtgagggagccagcagctctgatggctatgtcgttggtgtggaagttggtatcaatcacaagtcgactgtcatacacaagacatgcatcattgagggctttaaacgtttcataatccacattcttctcacagaagctgaagaacatagagcactggagtctgaaaggcttggtgggtgtggtgaaggaggcgctgtagatggggtctgggtgcaggccgtcattccactgggccaggatcgcatcccggtacatagtgactccggcggctcctagcgcgtccgccacggcgctctccaccgagtagttgttgatgcaggtgatggtggaggcgggcgggggctgcacgaggtggatgcggctgccgctcacgccaaggtttaagagcgtctccacggtggtgtaagtatcaattgtattcccatagacaatgatattcccttctgtggtgatggagttattccttatccaaatcagtgccttaaagcaatcctcttcctcgttgagagtgaaatggttgcaaggaactttccccgtgtaccgccgctgactgctgttgggaacctccctgtttgtcaggtgttgactaatatcagcctctgtagggcatgggacctggtactgctgcccggtgcagaggatgaggtggtcgtagggcacgatctcgtccgtggaaagcacaacgtgcttggctgctcggtctatgccggtcattctacccaccacgacattaacccaggagcacagtgacatcagtgcataatctttatcattaaaacagtggtcgctggctaaaaatttcctttgttcagtgtccagaagtttttttcctgggagtccatgagttgaaatcagggtaagattattaaacttcatgtgagagcaaaataccaatgtctctaggaaggaaattccaacactggatgcaccaaccacaatgatcttggcattgacagtaattttaggttccaatgttagttttctgtttgtatggtttaaagcataactcatcggatccttggagaccgcctttgatggagcgtttatgccaagcttttccagaggatagacaatctgtcgtcgtggtcgcacgggaaccaagtaatgaagggcagatgtcagggagtgggcgtaggggttctggaactgaaagacagcaatcttgccttctctggattttgggtaaacacggtagtagagacaggatttaaagcctaaacgcaggatctccttcagaaagaacttggtgtagtgccggaaaatggggttgagggcaaagtgatgcatgtgcccgtgttcttcgcgctggtggtgactgaagtagatgaaatcttcaatgttgtaatgggaccgtatgtactcaatgtccatttcatttctgatcactgcaataccaactatttgttctgcaacttcagctacaaatgcctgcagcagtgttccatcagggtctttgcgagccttgttgtaacggtctaagtcctccaatatgcttttattcaacatgagggtgctgacaagattttccacaccaggagtatccaagagagtggcaaatcttatattaatggacttgagcaatccagcccggtggaagacgtagaggtcctgctcgagggtgcaggtgttgaaagggaccattttcacgaagttctggatgaggaagaactcgggggtgagatggggcagagaaattacacagaagttcttatcagaaaaaagactgaaaacaaaattcataaaatccagcgaccttgcttcatatttctcatcaatacaaaacagctgaatacaaaaagcagctgaggctcccctgtagatggggcggaagtggacgggctcttcaggcagtacgagcgatgccaagctcctactgctgacatggtgatactgtgcatatccagtggagatgtcactgagtttttctatgtcctccggttcactaacatttccactttggactgctgttaaagcttcctcggatgcagcttctctggcaatatttccctggatgttttccatggtatctggagagacaggttcctgcaactcctcgactattttttgggaaccttggctgctactcctgagctcagcatcttgacttcttcggacacttaggtcttgtggtgattccagaacgtcatcaggatgtgggaaacagagtccgtggaaagggcccaagtcaaagcactcatgcagcagttgcatgttcactcttgagcacacactcatgaacccaacagctgtgccttccacctcacacacaacagcatgattctcttcatcttgggcctctattagttcggccaggaagtattcaccgtaagtttccttcagaattgtgtcatagcgcataaatattggcatgagatcgtcatggtcttccaccctggctttgcgaacgtgcagctgaggatagtggctgtgcctgtgacatatatgcactgcaaagtcttcctcatacgtcagacacgggatgttccccacttggtcaaaaacagttatgagagttgagcctaggctcatgtaggatggcacgatgagaaatatgaagtgcagctctggcactgccttatacacggttcgaagaatctctttgcaacagccaacagaatactcatccacggccacaaagaggtgcatgaacaacgtattcaggggtgtgcatgggatgtcactgtcgagctcccggaacactgacacccagtcatcctgcttggcaacattccagttggggtagtccaggaaggtggcctgggccatgatctcctccttgtcattgcagagggtaacagcaaggttggccttttctctcatccgcagctccaggacgccgcactccacgcgctgccgcaaggaggacgcgcagcctggtcaccatggaaacggt

SEQ ID NO: 16714 - RNA, 3696 nt, Homo sapiens
  source 1..3696: mol_type = other RNA
taaagtgcttatagtgcaggtagtcaagagtgcttctctccaccagggttttgtagatggattcctcaaaaactcttttgaggtattgcctgggcttctcagtcgggttgatttcctcatcttctatttgatgggctaactgctctatggaaggaagatcttcctcctccttggaggctaagatttggcgtaactctttcctgagatcaataaaacgatcgtggaacagggccaggcaccacggctcggtgaagtagctatagagatctgtgatcaggttttcatcgtaccgagcacacaggttgttgaggagttgctcgtgctggccaaacaagcggatgtagttggaggcggggaagggctccctagaaaggcacgtgatggtttccaccattttatacttgttaatatgaattcggaagtaagtcccatttttcgcactgccggttactagttctaaaccataattaggctgtgccatttgtacctccaagggagttggaatggcaggcttggcaatatgcagataatggtaagacccaggaagaatgcccccttgaatcttggctcccttgtacatggggatgagccggtcaagattagctggtggctcggtcacaggctcaagggttggatcaaagagatgtagcatagctgctgccagctgaaagccaatttctttggaactgaagttgctgtgagtccactcatttgagtagtatctattggagaatttggtgagggagccagcagctctgatggctatgtcgttggtgtggaagttggtatcaatcacaagtcgactgtcatacacaagacatgcatcattgagggctttaaacgtttcataatccacattcttctcacagaagctgaagaacatagagcactggagtctgaaaggcttggtgggtgtggtgaaggaggcgctgtagatggggtctgggtgcaggccgtcattccactgggccaggatcgcatcccggtacatagtgactccggcggctcctagcgcgtccgccacggcgctctccaccgagtagttgttgatgcaggtgatggtggaggcgggcgggggctgcacgaggtggatgcggctgccgctcacgccaaggtttaagagcgtctccacggtggtgtaagtatcaattgtattcccatagacaatgatattcccttctgtggtgatggagttattccttatccaaatcagtgccttaaagcaatcctcttcctcgttgagagtgaaatggttgcaaggaactttccccgtgtaccgccgctgactgctgttgggaacctccctgtttgtcaggtgttgactaatatcagcctctgtagggcatgggacctggtactgctgcccggtgcagaggatgaggtggtcgtagggcacgatctcgtccgtggaaagcacaacgtgcttggctgctcggtctatgccggtcattctacccaccacgacattaacccaggagcacagtgacatcagtgcataatctttatcattaaaacagtggtcgctggctaaaaatttcctttgttcagtgtccagaagtttttttcctgggagtccatgagttgaaatcagggtaagattattaaacttcatgtgagagcaaaataccaatgtctctaggaaggaaattccaacactggatgcaccaaccacaatgatcttggcattgacagtaattttaggttccaatgttagttttctgtttgtatggtttaaagcataactcatcggatccttggagaccgcctttgatggagcgtttatgccaagcttttccagaggatagacaatctgtcgtcgtggtcgcacgggaaccaagtaatgaagggcagatgtcagggagtgggcgtaggggttctggaactgaaagacagcaatcttgccttctctggattttgggtaaacacggtagtagagacaggatttaaagcctaaacgcaggatctccttcagaaagaacttggtgtagtgccggaaaatggggttgagggcaaagtgatgcatgtgcccgtgttcttcgcgctggtggtgactgaagtagatgaaatcttcaatgttgtaatgggaccgtatgtactcaatgtccatttcatttctgatcactgcaataccaactatttgttctgcaacttcagctacaaatgcctgcagcagtgttccatcagggtctttgcgagccttgttgtaacggtctaagtcctccaatatgcttttattcaacatgagggtgctgacaagattttccacaccaggagtatccaagagagtggcaaatcttatattaatggacttgagcaatccagcccggtggaagacgtagaggtcctgctcgagggtgcaggtgttgaaagggaccattttcacgaagttctggatgaggaagaactcgggggtgagatggggcagagaaattacacagaagttcttatcagaaaaaagactgaaaacaaaattcataaaatccagcgaccttgcttcatatttctcatcaatacaaaacagctgaatacaaaaagcagctgaggctcccctgtagatggggcggaagtggacgggctcttcaggcagtacgagcgatgccaagctcctactgctgacatggtgatactgtgcatatccagtggagatgtcactgagtttttctatgtcctggatgttttccatggtatctggagagacaggttcctgcaactcctcgactattttttgggaaccttggctgctactcctgagctcagcatcttgacttcttcggacacttaggtcttgtggtgattccagaacgtcatcaggatgtgggaaacagagtccgtggaaagggcccaagtcaaagcactcatgcagcagttgcatgttcactcttgagcacacactcatgaacccaacagctgtgccttccacctcacacacaacagcatgattctcttcatcttgggcctctattagttcggccaggaagtattcaccgtaagtttccttcagaattgtgtcatagcgcataaatattggcatgagatcgtcatggtcttccaccctggctttgcgaacgtgcagctgaggatagtggctgtgcctgtgacatatatgcactgcaaagtcttcctcatacgtcagacacgggatgttccccacttggtcaaaaacagttatgagagttgagcctaggctcatgtaggatggcacgatgagaaatatgaagtgcagctctggcactgccttatacacggttcgaagaatctctttgcaacagccaacagaatactcatccacggccacaaagaggtgcatgaacaacgtattcaggggtgtgcatgggatgtcactgtcgagctcccggaacactgacacccagtcatcctgcttggcaacattccagttggggtagtccaggaaggtggcctgggccatgatctcctccttgtcattgcagagggtaacagcaaggttggccttttctagaagatagatgatatttagcttcccaaacagcttgcaggtaaattttctaataaggcttttgatacaataaacatcctgtgattctgttcttcggcaatgaacaacttctacctttcctcttggagaagtgagtactgacattttttatcctcatccgcagctccaggacgccgcactccacgcgctgccgcaaggaggacgcgcagcctggtcaccat

SEQ ID NO: 16715 - RNA, 3490 nt, Homo sapiens
  source 1..3490: mol_type = other RNA
taaagtgcttatagtgcaggtagtcaagagtgcttctctccaccagggttttgtagatggattcctcaaaaactcttttgaggtattgcctgggcttctcagtcgggttgatttcctcatcttctatttgatgggctaactgctctatggaaggaagatcttcctcctccttggaggctaagatttggcgtaactctttcctgagatcaataaaacgatcgtggaacagggccaggcaccacggctcggtgaagtagctatagagatctgtgatcaggttttcatcgtaccgagcacacaggttgttgaggagttgctcgtgctggccaaacaagcggatgtagttggaggcggggaagggctccctagaaaggcacgtgatggtttccaccattttatacttgttaatatgaattcggaagtaagtcccatttttcgcactgccggttactagttctaaaccataattaggctgtgccatttgtacctccaagggagttggaatggcaggcttggcaatatgcagataatggtaagacccaggaagaatgcccccttgaatcttggctcccttgtacatggggatgagccggtcaagattagctggtggctcggtcacaggctcaagggttggatcaaagagatgtagcatagctgctgccagctgaaagccaatttctttggaactgaagttgctgtgagtccactcatttgagtagtatctattggagaatttggtgagggagccagcagctctgatggctatgtcgttggtgtggaagttggtatcaatcacaagtcgactgtcatacacaagacatgcatcattgagggctttaaacgtttcataatccacattcttctcacagaagctgaagaacatagagcactggagtctgaaaggcttggtgggtgtggtgaaggaggcgctgtagatggggtctgggtgcaggccgtcattccactgggccaggatcgcatcccggtacatagtgactccggcggctcctagcgcgtccgccacggcgctctccaccgagtagttgttgatgcaggtgatggtggaggcgggcgggggctgcacgaggtggatgcggctgccgctcacgccaaggtttaagagcgtctccacggtggtgtaagtatcaattgtattcccatagacaatgatattcccttctgtggtgatggagttattccttatccaaatcagtgccttaaagcaatcctcttcctcgttgagagtgaaatggttgcaaggaactttccccgtgtaccgccgctgactgctgttgggaacctccctgtttgtcaggtgttgactaatatcagcctctgtagggcatgggacctggtactgctgcccggtgcagaggatgaggtggtcgtagggcacgatctcgtccgtggaaagcacaacgtgcttggctgctcggtctatgccggtcattctacccaccacgacattaacccaggagcacagtgacatcagtgcataatctttatcattaaaacagtggtcgctggctaaaaatttcctttgttcagtgtccagaagtttttttcctgggagtccatgagttgaaatcagggtaagattattaaacttcatgtgagagcaaaataccaatgtctctaggaaggaaattccaacactggatgcaccaaccacaatgatcttggcattgacagtaattttaggttccaatgttagttttctgtttgtatggtttaaagcataactcatcggatccttggagaccgcctttgatggagcgtttatgccaagcttttccagaggatagacaatctgtcgtcgtggtcgcacgggaaccaagtaatgaagggcagatgtcagggagtgggcgtaggggttctggaacttgccttctctggattttgggtaaacacggtagtagagacaggatttaaagcctaaacgcaggatctccttcagaaagaacttggtgtagtgccggaaaatggggttgagggcaaagtgatgcatgtgcccgtgttcttcgcgctggtggtgactgaagtagatgaaatcttcaatgttgtaatgggaccgtatgtactcaatgtcagggtctttgcgagccttgttgtaacggtctaagtcctccaatatgcttttattcaacatgagggtgctgacaagattttccacaccaggagtatccaagagagtggcaaatcttatattaatggacttgagcaatccagcccggtggaagacgtagaggtcctgctcgagggtgcaggtgttgaaagggaccattttcacgaagttctggatgaggaagaactcgggggtgagatggggcagagaaattacacagaagttcttatcagaaaaaagactgaaaacaaaattcataaaatccagcgacctccggttcactaacatttccactttggactgctgttaaagcttcctcggatgcagcttctctggcaatatttccctggatgttttccatggtatctggagagacaggttcctgcaactcctcgactattttttgggaaccttggctgctactcctgagctcagcatcttgacttcttcggacacttaggtcttgtggtgattccagaacgtcatcaggatgtgggaaacagagtccgtggaaagggcccaagtcaaagcactcatgcagcagttgcatgttcactcttgagcacacactcatgaacccaacagctgtgccttccacctcacacacaacagcatgattctcttcatcttgggcctctattagttcggccaggaagtattcaccgtaagtttccttcagaattgtgtcatagcgcataaatattggcatgagatcgtcatggtcttccaccctggctttgcgaacgtgcagctgaggatagtggctgtgcctgtgacatatatgcactgcaaagtcttcctcatacgtcagacacgggatgttccccacttggtcaaaaacagttatgagagttgagcctaggctcatgtaggatggcacgatgagaaatatgaagtgcagctctggcactgccttatacacggttcgaagaatctctttgcaacagccaacagaatactcatccacggccacaaagaggtgcatgaacaacgtattcaggggtgtgcatgggatgtcactgtcgagctcccggaacactgacacccagtcatcctgcttggcaacattccagttggggtagtccaggaaggtggcctgggccatgatctcctccttgtcattgcagagggtaacagcaaggttggccttttctagaagatagatgatatttagcttcccaaacagcttgcaggtaaattttctaataaggcttttgatacaataaacatcctgtgattctgttcttcggcaatgaacaacttctacctttcctcttggagaagtgagtactgacattttttatcctcatccgcagctccaggacgccgcactccacgcgctgccgcaaggaggacgcgcagcct

SEQ ID NO: 16716 - RNA, 2626 nt, Homo sapiens
  source 1..2626: mol_type = other RNA
taaagtgcttatagtgcaggtagtcaagagtgcttctctccaccagggttttgtagatggattcctcaaaaactcttttgaggtattgcctgggcttctcagtcgggttgatttcctcatcttctatttgatgggctaactgctctatggaaggaagatcttcctcctccttggaggctaagatttggcgtaactctttcctgagatcaataaaacgatcgtggaacagggccaggcaccacggctcggtgaagtagctatagagatctgtgatcaggttttcatcgtaccgagcacacaggttgttgaggagttgctcgtgctggccaaacaagcggatgtagttggaggcggggaagggctccctagaaaggcacgtgatggtttccaccattttatacttgttaatatgaattcggaagtaagtcccatttttcgcactgccggttactagttctaaaccataattaggctgtgccatttgtacctccaagggagttggaatggcaggcttggcaatatgcagataatggtaagacccaggaagaatgcccccttgaatcttggctcccttgtacatggggatgagccggtcaagattagctggtggctcggtcacaggctcaagggttggatcaaagagatgtagcatagctgctgccagctgaaagccaatttctttggaactgaagttgctgtgagtccactcatttgagtagtatctattggagaatttggtgagggagccagcagctctgatggctatgtcgttggtgtggaagttggtatcaatcacaagtcgactgtcatacacaagacatgcatcattgagggctttaaacgtttcataatccacattcttctcacagaagctgaagaacatagagcactggagtctgaaaggcttggtgggtgtggtgaaggaggcgctgtagatggggtctgggtgcaggccgtcattccactgggccaggatcgcatcccggtacatagtgactccggcggctcctagcgcgtccgccacggcgctctccaccgagtagttgttgatgcaggtgatggtggaggcgggcgggggctgcacgaggtggatgcggctgccgctcacgccaaggtttaagagcgtctccacggtggtgtaagtatcaattgtattcccatagacaatgatattcccttctgtggtgatggagttattccttatccaaatcagtgccttaaagcaatcctcttcctcgttgagagtgaaatggttgcaaggaactttccccgtgtaccgccgctgactgctgttgggaacctccctgtttgtcaggtgttgactaatatcagcctctgtagggcatgggacctggtactgctgcccggtgcagaggatgaggtggtcgtagggcacgatctcgtccgtggaaagcacaacgtgcttggctgctcggtctatgccggtcattctacccaccacgacattaacccaggagcacagtgacatcagtgcataatctttatcattaaaacagtggtcgctggctaaaaatttcctttgttcagtgtccagaagtttttttcctgggagtccatgagttgaaatcagggtaagattattaaacttcatgtgagagcaaaataccaatgtctctaggaaggaaattccaacactggatgcaccaaccacaatgatcttggcattgacagtaattttaggttccaatgttagttttctgtttgtatggtttaaagcataactcatcggatccttggagaccgcctttgatggagcgtttatgccaagcttttccagaggatagacaatctgtcgtcgtggtcgcacgggaaccaagtaatgaagggcagatgtcagggagtgggcgtaggggttctggaacttgccttctctggattttgggtaaacacggtagtagagacaggatttaaagcctaaacgcaggatctccttcagaaagaacttggtgtagtgccggaaaatggggttgagggcaaagtgatgcatgtgcccgtgttcttcgcgctggtggtgactgaagtagatgaaatcttcaatgttgtaatgggaccgtatgtactcaatgtcagggtctttgcgagccttgttgtaacggtctaagtcctccaatatgcttttattcaacatgagggtgctgacaagattttccacaccaggagtatccaagagagtggcaaatcttatattaatggacttgagcaatccagcccggtggaagacgtagaggtcctgctcgagggtgcaggtgttgaaagggaccattttcacgaagttctggatgaggaagaactcgggggtgagatggggcagagaaattacacagaagttcttatcagaaaaaagactgaaaacaaaattcataaaatccagcgacctggatgttttccatggtatctggagagacaggttcctgcaactcctcgactattttttgggaaccttggctgctactcctgagctcagcatcttgacttcttcggacacttaggtcttgtggtgattccagaacgtcatcaggatgtgggaaacagagtccgtggaaagggcccaagtcaaagcactcatgcagcagttgcatgttcactcttgagcacacactcatga

SEQ ID NO: 16717 - RNA, 3678 nt, Homo sapiens
  source 1..3678: mol_type = other RNA
taaagtgcttatagtgcaggtagtcaagagtgcttctctccaccagggttttgtagatggattcctcaaaaactcttttgaggtattgcctgggcttctcagtcgggttgatttcctcatcttctatttgatgggctaactgctctatggaaggaagatcttcctcctccttggaggctaagatttggcgtaactctttcctgagatcaataaaacgatcgtggaacagggccaggcaccacggctcggtgaagtagctatagagatctgtgatcaggttttcatcgtaccgagcacacaggttgttgaggagttgctcgtgctggccaaacaagcggatgtagttggaggcggggaagggctccctagaaaggcacgtgatggtttccaccattttatacttgttaatatgaattcggaagtaagtcccatttttcgcactgccggttactagttctaaaccataattaggctgtgccatttgtacctccaagggagttggaatggcaggcttggcaatatgcagataatggtaagacccaggaagaatgcccccttgaatcttggctcccttgtacatggggatgagccggtcaagattagctggtggctcggtcacaggctcaagggttggatcaaagagatgtagcatagctgctgccagctgaaagccaatttctttggaactgaagttgctgtgagtccactcatttgagtagtatctattggagaatttggtgagggagccagcagctctgatggctatgtcgttggtgtggaagttggtatcaatcacaagtcgactgtcatacacaagacatgcatcattgagggctttaaacgtttcataatccacattcttctcacagaagctgaagaacatagagcactggagtctgaaaggcttggtgggtgtggtgaaggaggcgctgtagatggggtctgggtgcaggccgtcattccactgggccaggatcgcatcccggtacatagtgactccggcggctcctagcgcgtccgccacggcgctctccaccgagtagttgttgatgcaggtgatggtggaggcgggcgggggctgcacgaggtggatgcggctgccgctcacgccaaggtttaagagcgtctccacggtggtgtaagtatcaattgtattcccatagacaatgatattcccttctgtggtgatggagttattccttatccaaatcagtgccttaaagcaatcctcttcctcgttgagagtgaaatggttgcaaggaactttccccgtgtaccgccgctgactgctgttgggaacctccctgtttgtcaggtgttgactaatatcagcctctgtagggcatgggacctggtactgctgcccggtgcagaggatgaggtggtcgtagggcacgatctcgtccgtggaaagcacaacgtgcttggctgctcggtctatgccggtcattctacccaccacgacattaacccaggagcacagtgacatcagtgcataatctttatcattaaaacagtggtcgctggctaaaaatttcctttgttcagtgtccagaagtttttttcctgggagtccatgagttgaaatcagggtaagattattaaacttcatgtgagagcaaaataccaatgtctctaggaaggaaattccaacactggatgcaccaaccacaatgatcttggcattgacagtaattttaggttccaatgttagttttctgtttgtatggtttaaagcataactcatcggatccttggagaccgcctttgatggagcgtttatgccaagcttttccagaggatagacaatctgtcgtcgtggtcgcacgggaaccaagtaatgaagggcagatgtcagggagtgggcgtaggggttctggaacttgccttctctggattttgggtaaacacggtagtagagacaggatttaaagcctaaacgcaggatctccttcagaaagaacttggtgtagtgccggaaaatggggttgagggcaaagtgatgcatgtgcccgtgttcttcgcgctggtggtgactgaagtagatgaaatcttcaatgttgtaatgggaccgtatgtactcaatgtcagggtctttgcgagccttgttgtaacggtctaagtcctccaatatgcttttattcaacatgagggtgctgacaagattttccacaccaggagtatccaagagagtggcaaatcttatattaatggacttgagcaatccagcccggtggaagacgtagaggtcctgctcgagggtgcaggtgttgaaagggaccattttcacgaagttctggatgaggaagaactcgggggtgagatggggcagagaaattacacagaagttcttatcagaaaaaagactgaaaacaaaattcataaaatccagcgaccttgcttcatatttctcatcaatacaaaacagctgaatacaaaaagcagctgaggctcccctgtagatggggcggaagtggacgggctcttcaggcagtacgagcgatgccaagctcctactgctgacatggtgatactgtgcatatccagtggagatgtcactgagtttttctatgtcctccggttcactaacatttccactttggactgctgttaaagcttcctcggatgcagcttctctggcaatatttccctggatgttttccatggtatctggagagacaggttcctgcaactcctcgactattttttgggaaccttggctgctactcctgagctcagcatcttgacttcttcggacacttaggtcttgtggtgattccagaacgtcatcaggatgtgggaaacagagtccgtggaaagggcccaagtcaaagcactcatgcagcagttgcatgttcactcttgagcacacactcatgaacccaacagctgtgccttccacctcacacacaacagcatgattctcttcatcttgggcctctattagttcggccaggaagtattcaccgtaagtttccttcagaattgtgtcatagcgcataaatattggcatgagatcgtcatggtcttccaccctggctttgcgaacgtgcagctgaggatagtggctgtgcctgtgacatatatgcactgcaaagtcttcctcatacgtcagacacgggatgttccccacttggtcaaaaacagttatgagagttgagcctaggctcatgtaggatggcacgatgagaaatatgaagtgcagctctggcactgccttatacacggttcgaagaatctctttgcaacagccaacagaatactcatccacggccacaaagaggtgcatgaacaacgtattcaggggtgtgcatgggatgtcactgtcgagctcccggaacactgacacccagtcatcctgcttggcaacattccagttggggtagtccaggaaggtggcctgggccatgatctcctccttgtcattgcagagggtaacagcaaggttggccttttctagaagatagatgatatttagcttcccaaacagcttgcaggtaaattttctaataaggcttttgatacaataaacatcctgtgattctgttcttcggcaatgaacaacttctacctttcctcttggagaagtgagtactgacattttttatcctcatccgcagctccaggacgccgcactccacgcgctgccgcaaggaggacgcgcagcctggtcaccat

SEQ ID NO: 16718 - RNA, 3696 nt, Homo sapiens
  source 1..3696: mol_type = other RNA
taaagtgcttatagtgcaggtagtcaagagtgcttctctccaccagggttttgtagatggattcctcaaaaactcttttgaggtattgcctgggcttctcagtcgggttgatttcctcatcttctatttgatgggctaactgctctatggaaggaagatcttcctcctccttggaggctaagatttggcgtaactctttcctgagatcaataaaacgatcgtggaacagggccaggcaccacggctcggtgaagtagctatagagatctgtgatcaggttttcatcgtaccgagcacacaggttgttgaggagttgctcgtgctggccaaacaagcggatgtagttggaggcggggaagggctccctagaaaggcacgtgatggtttccaccattttatacttgttaatatgaattcggaagtaagtcccatttttcgcactgccggttactagttctaaaccataattaggctgtgccatttgtacctccaagggagttggaatggcaggcttggcaatatgcagataatggtaagacccaggaagaatgcccccttgaatcttggctcccttgtacatggggatgagccggtcaagattagctggtggctcggtcacaggctcaagggttggatcaaagagatgtagcatagctgctgccagctgaaagccaatttctttggaactgaagttgctgtgagtccactcatttgagtagtatctattggagaatttggtgagggagccagcagctctgatggctatgtcgttggtgtggaagttggtatcaatcacaagtcgactgtcatacacaagacatgcatcattgagggctttaaacgtttcataatccacattcttctcacagaagctgaagaacatagagcactggagtctgaaaggcttggtgggtgtggtgaaggaggcgctgtagatggggtctgggtgcaggccgtcattccactgggccaggatcgcatcccggtacatagtgactccggcggctcctagcgcgtccgccacggcgctctccaccgagtagttgttgatgcaggtgatggtggaggcgggcgggggctgcacgaggtggatgcggctgccgctcacgccaaggtttaagagcgtctccacggtggtgtaagtatcaattgtattcccatagacaatgatattcccttctgtggtgatggagttattccttatccaaatcagtgccttaaagcaatcctcttcctcgttgagagtgaaatggttgcaaggaactttccccgtgtaccgccgctgactgctgttgggaacctccctgtttgtcaggtgttgactaatatcagcctctgtagggcatgggacctggtactgctgcccggtgcagaggatgaggtggtcgtagggcacgatctcgtccgtggaaagcacaacgtgcttggctgctcggtctatgccggtcattctacccaccacgacattaacccaggagcacagtgacatcagtgcataatctttatcattaaaacagtggtcgctggctaaaaatttcctttgttcagtgtccagaagtttttttcctgggagtccatgagttgaaatcagggtaagattattaaacttcatgtgagagcaaaataccaatgtctctaggaaggaaattccaacactggatgcaccaaccacaatgatcttggcattgacagtaattttaggttccaatgttagttttctgtttgtatggtttaaagcataactcatcggatccttggagaccgcctttgatggagcgtttatgccaagcttttccagaggatagacaatctgtcgtcgtggtcgcacgggaaccaagtaatgaagggcagatgtcagggagtgggcgtaggggttctggaacttgccttctctggattttgggtaaacacggtagtagagacaggatttaaagcctaaacgcaggatctccttcagaaagaacttggtgtagtgccggaaaatggggttgagggcaaagtgatgcatgtgcccgtgttcttcgcgctggtggtgactgaagtagatgaaatcttcaatgttgtaatgggaccgtatgtactcaatgtccatttcatttctgatcactgcaataccaactatttgttctgcaacttcagctacaaatgcctgcagcagtgttccatcagggtctttgcgagccttgttgtaacggtctaagtcctccaatatgcttttattcaacatgagggtgctgacaagattttccacaccaggagtatccaagagagtggcaaatcttatattaatggacttgagcaatccagcccggtggaagacgtagaggtcctgctcgagggtgcaggtgttgaaagggaccattttcacgaagttagaaaaaagactgaaaacaaaattcataaaatccagcgaccttgcttcatatttctcatcaatacaaaacagctgaatacaaaaagcagctgaggctcccctgtagatggggcggaagtggacgggctcttcaggcagtacgagcgatgccaagctcctactgctgacatggtgatactgtgcatatccagtggagatgtcactgagtttttctatgtcctccggttcactaacatttccactttggactgctgttaaagcttcctcggatgcagcttctctggcaatatttccctggatgttttccatggtatctggagagacaggttcctgcaactcctcgactattttttgggaaccttggctgctactcctgagctcagcatcttgacttcttcggacacttaggtcttgtggtgattccagaacgtcatcaggatgtgggaaacagagtccgtggaaagggcccaagtcaaagcactcatgcagcagttgcatgttcactcttgagcacacactcatgaacccaacagctgtgccttccacctcacacacaacagcatgattctcttcatcttgggcctctattagttcggccaggaagtattcaccgtaagtttccttcagaattgtgtcatagcgcataaatattggcatgagatcgtcatggtcttccaccctggctttgcgaacgtgcagctgaggatagtggctgtgcctgtgacatatatgcactgcaaagtcttcctcatacgtcagacacgggatgttccccacttggtcaaaaacagttatgagagttgagcctaggctcatgtaggatggcacgatgagaaatatgaagtgcagctctggcactgccttatacacggttcgaagaatctctttgcaacagccaacagaatactcatccacggccacaaagaggtgcatgaacaacgtattcaggggtgtgcatgggatgtcactgtcgagctcccggaacactgacacccagtcatcctgcttggcaacattccagttggggtagtccaggaaggtggcctgggccatgatctcctccttgtcattgcagagggtaacagcaaggttggccttttctagaagatagatgatatttagcttcccaaacagcttgcaggtaaattttctaataaggcttttgatacaataaacatcctgtgattctgttcttcggcaatgaacaacttctacctttcctcttggagaagtgagtactgacattttttatcctcatccgcagctccaggacgccgcactccacgcgctgccgcaaggaggacgcgcagcctggtcaccat

SEQ ID NO: 16719 - RNA, 3756 nt, Homo sapiens
  source 1..3756: mol_type = other RNA
taaagtgcttatagtgcaggtagtcaagagtgcttctctccaccagggttttgtagatggattcctcaaaaactcttttgaggtattgcctgggcttctcagtcgggttgatttcctcatcttctatttgatgggctaactgctctatggaaggaagatcttcctcctccttggaggctaagatttggcgtaactctttcctgagatcaataaaacgatcgtggaacagggccaggcaccacggctcggtgaagtagctatagagatctgtgatcaggttttcatcgtaccgagcacacaggttgttgaggagttgctcgtgctggccaaacaagcggatgtagttggaggcggggaagggctccctagaaaggcacgtgatggtttccaccattttatacttgttaatatgaattcggaagtaagtcccatttttcgcactgccggttactagttctaaaccataattaggctgtgccatttgtacctccaagggagttggaatggcaggcttggcaatatgcagataatggtaagacccaggaagaatgcccccttgaatcttggctcccttgtacatggggatgagccggtcaagattagctggtggctcggtcacaggctcaagggttggatcaaagagatgtagcatagctgctgccagctgaaagccaatttctttggaactgaagttgctgtgagtccactcatttgagtagtatctattggagaatttggtgagggagccagcagctctgatggctatgtcgttggtgtggaagttggtatcaatcacaagtcgactgtcatacacaagacatgcatcattgagggctttaaacgtttcataatccacattcttctcacagaagctgaagaacatagagcactggagtctgaaaggcttggtgggtgtggtgaaggaggcgctgtagatggggtctgggtgcaggccgtcattccactgggccaggatcgcatcccggtacatagtgactccggcggctcctagcgcgtccgccacggcgctctccaccgagtagttgttgatgcaggtgatggtggaggcgggcgggggctgcacgaggtggatgcggctgccgctcacgccaaggtttaagagcgtctccacggtggtgtaagtatcaattgtattcccatagacaatgatattcccttctgtggtgatggagttattccttatccaaatcagtgccttaaagcaatcctcttcctcgttgagagtgaaatggttgcaaggaactttccccgtgtaccgccgctgactgctgttgggaacctccctgtttgtcaggtgttgactaatatcagcctctgtagggcatgggacctggtactgctgcccggtgcagaggatgaggtggtcgtagggcacgatctcgtccgtggaaagcacaacgtgcttggctgctcggtctatgccggtcattctacccaccacgacattaacccaggagcacagtgacatcagtgcataatctttatcattaaaacagtggtcgctggctaaaaatttcctttgttcagtgtccagaagtttttttcctgggagtccatgagttgaaatcagggtaagattattaaacttcatgtgagagcaaaataccaatgtctctaggaaggaaattccaacactggatgcaccaaccacaatgatcttggcattgacagtaattttaggttccaatgttagttttctgtttgtatggtttaaagcataactcatcggatccttggagaccgcctttgatggagcgtttatgccaagcttttccagaggatagacaatctgtcgtcgtggtcgcacgggaaccaagtaatgaagggcagatgtcagggagtgggcgtaggggttctggaacttgccttctctggattttgggtaaacacggtagtagagacaggatttaaagcctaaacgcaggatctccttcagaaagaacttggtgtagtgccggaaaatggggttgagggcaaagtgatgcatgtgcccgtgttcttcgcgctggtggtgactgaagtagatgaaatcttcaatgttgtaatgggaccgtatgtactcaatgtccatttcatttctgatcactgcaataccaactatttgttctgcaacttcagctacaaatgcctgcagcagtgttccatcagggtctttgcgagccttgttgtaacggtctaagtcctccaatatgcttttattcaacatgagggtgctgacaagattttccacaccaggagtatccaagagagtggcaaatcttatattaatggacttgagcaatccagcccggtggaagacgtagaggtcctgctcgagggtgcaggtgttgaaagggaccattttcacgaagttctggatgaggaagaactcgggggtgagatggggcagagaaattacacagaagttcttatcagaaaaaagactgaaaacaaaattcataaaatccagcgaccttgcttcatatttctcatcaatacaaaacagctgaatacaaaaagcagctgaggctcccctgtagatggggcggaagtggacgggctcttcaggcagtacgagcgatgccaagctcctactgctgacatggtgatactgtgcatatccagtggagatgtcactgagtttttctatgtcctccggttcactaacatttccactttggactgctgttaaagcttcctcggatgcagcttctctggcaatatttccctggatgttttccatggtatctggagagacaggttcctgcaactcctcgactattttttgggaaccttggctgctactcctgagctcagcatcttgacttcttcggacacttaggtcttgtggtgattccagaacgtcatcaggatgtgggaaacagagtccgtggaaagggcccaagtcaaagcactcatgcagcagttgcatgttcactcttgagcacacactcatgaacccaacagctgtgccttccacctcacacacaacagcatgattctcttcatcttgggcctctattagttcggccaggaagtattcaccgtaagtttccttcagaattgtgtcatagcgcataaatattggcatgagatcgtcatggtcttccaccctggctttgcgaacgtgcagctgaggatagtggctgtgcctgtgacatatatgcactgcaaagtcttcctcatacgtcagacacgggatgttccccacttggtcaaaaacagttatgagagttgagcctaggctcatgtaggatggcacgatgagaaatatgaagtgcagctctggcactgccttatacacggttcgaagaatctctttgcaacagccaacagaatactcatccacggccacaaagaggtgcatgaacaacgtattcaggggtgtgcatgggatgtcactgtcgagctcccggaacactgacacccagtcatcctgcttggcaacattccagttggggtagtccaggaaggtggcctgggccatgatctcctccttgtcattgcagagggtaacagcaaggttggccttttctagaagatagatgatatttagcttcccaaacagcttgcaggtaaattttctaataaggcttttgatacaataaacatcctgtgattctgttcttcggcaatgaacaacttctacctttcctcttggagaagtgagtactgacattttttatcctcatccgcagctccaggacgccgcactccacgcgctgccgcaaggaggacgcgcagcctggtcaccat

SEQ ID NO: 16720 - RNA, 3775 nt, Homo sapiens
  source 1..3775: mol_type = other RNA
taaagtgcttatagtgcaggtagtcaagagtgcttctctccaccagggttttgtagatggattcctcaaaaactcttttgaggtattgcctgggcttctcagtcgggttgatttcctcatcttctatttgatgggctaactgctctatggaaggaagatcttcctcctccttggaggctaagatttggcgtaactctttcctgagatcaataaaacgatcgtggaacagggccaggcaccacggctcggtgaagtagctatagagatctgtgatcaggttttcatcgtaccgagcacacaggttgttgaggagttgctcgtgctggccaaacaagcggatgtagttggaggcggggaagggctccctagaaaggcacgtgatggtttccaccattttatacttgttaatatgaattcggaagtaagtcccatttttcgcactgccggttactagttctaaaccataattaggctgtgccatttgtacctccaagggagttggaatggcaggcttggcaatatgcagataatggtaagacccaggaagaatgcccccttgaatcttggctcccttgtacatggggatgagccggtcaagattagctggtggctcggtcacaggctcaagggttggatcaaagagatgtagcatagctgctgccagctgaaagccaatttctttggaactgaagttgctgtgagtccactcatttgagtagtatctattggagaatttggtgagggagccagcagctctgatggctatgtcgttggtgtggaagttggtatcaatcacaagtcgactgtcatacacaagacatgcatcattgagggctttaaacgtttcataatccacattcttctcacagaagctgaagaacatagagcactggagtctgaaaggcttggtgggtgtggtgaaggaggcgctgtagatggggtctgggtgcaggccgtcattccactgggccaggatcgcatcccggtacatagtgactccggcggctcctagcgcgtccgccacggcgctctccaccgagtagttgttgatgcaggtgatggtggaggcgggcgggggctgcacgaggtggatgcggctgccgctcacgccaaggtttaagagcgtctccacggtggtgtaagtatcaattgtattcccatagacaatgatattcccttctgtggtgatggagttattccttatccaaatcagtgccttaaagcaatcctcttcctcgttgagagtgaaatggttgcaaggaactttccccgtgtaccgccgctgactgctgttgggaacctccctgtttgtcaggtgttgactaatatcagcctctgtagggcatgggacctggtactgctgcccggtgcagaggatgaggtggtcgtagggcacgatctcgtccgtggaaagcacaacgtgcttggctgctcggtctatgccggtcattctacccaccacgacattaacccaggagcacagtgacatcagtgcataatctttatcattaaaacagtggtcgctggctaaaaatttcctttgttcagtgtccagaagtttttttcctgggagtccatgagttgaaatcagggtaagattattaaacttcatgtgagagcaaaataccaatgtctctaggaaggaaattccaacactggatgcaccaaccacaatgatcttggcattgacagtaattttaggttccaatgttagttttctgtttgtatggtttaaagcataactcatcggatccttggagaccgcctttgatggagcgtttatgccaagcttttccagaggatagacaatctgtcgtcgtggtcgcacgggaaccaagtaatgaagggcagatgtcagggagtgggcgtaggggttctggaacttgccttctctggattttgggtaaacacggtagtagagacaggatttaaagcctaaacgcaggatctccttcagaaagaacttggtgtagtgccggaaaatggggttgagggcaaagtgatgcatgtgcccgtgttcttcgcgctggtggtgactgaagtagatgaaatcttcaatgttgtaatgggaccgtatgtactcaatgtccatttcatttctgatcactgcaataccaactatttgttctgcaacttcagctacaaatgcctgcagcagtgttccatcagggtctttgcgagccttgttgtaacggtctaagtcctccaatatgcttttattcaacatgagggtgctgacaagattttccacaccaggagtatccaagagagtggcaaatcttatattaatggacttgagcaatccagcccggtggaagacgtagaggtcctgctcgagggtgcaggtgttgaaagggaccattttcacgaagttctggatgaggaagaactcgggggtgagatggggcagagaaattacacagaagttcttatcagaaaaaagactgaaaacaaaattcataaaatccagcgaccttgcttcatatttctcatcaatacaaaacagctgaatacaaaaagcagctgaggctcccctgtagatggggcggaagtggacgggctcttcaggcagtacgagcgatgccaagctcctactgctgacatggtgatactgtgcatatccagtggagatgtcactgagtttttctatgtcctccggttcactaacatttccactttggactgctgttaaagcttcctcggatgcagcttctctggcaatatttccctggatgttttccatggtatctggagagacaggttcctgcaactcctcgactattttttgggaaccttggctgctactcctgagctcagcatcttgacttcttcggacacttaggtcttgtggtgattccagaacgtcatcaggatgtgggaaacagagtccgtggaaagggcccaagtcaaagcactcatgcagcagttgcatgttcactcttgagcacacactcatgaacccaacagctgtgccttccacctcacacacaacagcatgattctcttcatcttgggcctctattagttcggccaggaagtattcaccgtaagtttccttcagaattgtgtcatagcgcataaatattggcatgagatcgtcatggtcttccaccctggctttgcgaacgtgcagctgaggatagtggctgtgcctgtgacatatatgcactgcaaagtcttcctcatacgtcagacacgggatgttccccacttggtcaaaaacagttatgagagttgagcctaggctcatgtaggatggcacgatgagaaatatgaagtgcagctctggcactgccttatacacggttcgaagaatctctttgcaacagccaacagaatactcatccacggccacaaagaggtgcatgaacaacgtattcaggggtgtgcatgggatgtcactgtcgagctcccggaacactgacacccagtcatcctgcttggcaacattccagttggggtagtccaggaaggtggcctgggccatgatctcctccttgtcattgcagagggtaacagcaaggttggccttttctagaagatagatgatatttagcttcccaaacagcttgcaggtaaattttctaataaggcttttgatacaataaacatcctgtgattctgttcttcggcaatgaacaacttctacctttcctcttggagaagtgagtactgacattttttatcctgtccccaaaagagagaaaaaagtccactcatccgcagctccaggacgccgcactccacgcgctgccgcaaggaggacgcgcagcct

SEQ ID NO: 16721 - RNA, 7015 nt, Homo sapiens
  source 1..7015: mol_type = other RNA
taaatttcacctttctgagaagaaaaacatgacttttcctaatgcacatagtttttcttaggtatctaaattagttgcttaaaagtaaaatgtacacttttatatgacacttaaagaaaattttgagttatagaaggagatgcttttataaaataaatgaacagccattctgtcttgacaataaaatccacaattctaagagataaaattgacacatatttccagatactaaatgtttggttttataagaaaaaagtattttgaagtaggcacagaggggttttacatgacaccaataagatatttactgtataaattgcaccactagacaaatacagctacaagaaaatcatttgaataagtcacacagctatcaaagcatctcacacattcattataattcactctttcatactagtttatatacactgagtgagtcattaaatattgcacttattggcccatgaaccctcaattctgaggtgttgaaaatagaaaacaaatctatttttataacatatttcatgcaacatttaagacatatcagttctacaaacaccattaaattgttgtacatttggacagtctaacggtatcacatcacgtctgacattaacaatatattaacaggaattacaggacagttttcctttagcacgtatcctagggataatgagacaatgcatggaaagccatcatattgatacagcaaacaatacccaaactttacttttacaagaagtatggaaccacttgacagatgtaagtcatgctcacgtccctgaaagggcaggtgtctgaggggctcaggtaccatctgtgtctgtaagaacagcattcacgaacctaagcaatacctagccccaaataacatgaatgcaaaataatttgcctcaagaaataaagccacagccaactctcacttgtccacgatgaaggaaatattaacacaggtgaatgaaatacacaggtaacctcaaacctcatttcagcaagtaatgactgtttgaaactccaccagtaatggttgctgatgggaagtaaatggtgaaatttgagtctcattttctattcttggtcctgtcattccatgaggatagtgttttgaaaaactgcagtaatttaaaagaaagtcagaaagtaaaagagaactgcaaatagaaagttcaatttgtccactagctagatggtctgatcttaacactcgagctctgagtgaggttttaaaatgactcatttctgttatctagaatgcttgcaaaatttatttcccctccactctctctgtttggaggaaattaattacatgcacagactaatcaaacgaaatcagtgtgaagaaccgattttatggaccttataagtaagatgtgagttatagctggaacatagtaaaagctcccttttccctagcactgagaaagcaccatagatggaattttgccttcttaaaaaaaagtatcagtgtttgcctgatacctttgtacaggcgagtgagcgtgtgagtgactgttgagaagggcagcactgtatgtgtaatctaaaagcaaatatttcaatctatcaaagggaaatattatttgaccggagtgtcaagcatttctgtaaatatttttaagaaaaaaattatttgtgaaataccagtaacaataggtagatacattttagataaatcccccaacttggtttttccctgttagggggtactatatttctacaacctagagccctttagatacagtgctgtgcaggggtaaaggcttttttattctggtcataaacttcatcttttacttaatttggcccagtaaattccatgatataaaacaggtttatgtctttaattgactttggtcaaaaattcacctaaaatatgaagaactcccaaaagctggctcaaaggttcagcatatcagaaagacttcaccattttacaggcaaactactaaagcgaaggtaatcaatgcacacaggcagagctgagcagagctgtagaggttgcattttccagggagtgacagaaaggccacatgggtgtagttgctcatgtggcacccggacagcacactaagtgactatacacgcaaaggaacagagttccgggttctagtcatgcaaactgtaattgtgagagaaagggttcttcagacggacaggccagctctgaagtatgccacaccaaaaataactgattgagcattccagtagtactatgaagattattaacaaacacacagtaactttttggtctagaagggttttagttatgacttttttataaataagattcatatcacagtttttcacatgcaggtgttacctacctcagcttggtatagcttggtagtttggatatgcttttaatatagtcccacaaatgccacactgttaactaaaatatcacatagtacatcctcaaccatgcactaagatacatgttggataaagcacatcacaatgaaccactgattatggactaccatgctctaaaattaatgttgcttcatggaagttcagttaatagtggaatgtatttaacttttaaaagagaagaagaaggttgtatatacccgaaagtctatcgtcagcatagatgtatttaaaattgaaagtttaaattggttccttaaaaaataaccagtgtactaaacaaaaggcctataattaatatgaataagatttaagtaggtgaaatatatatatttgtttactgagtgttttgatgtcttgtataatttgggttgtaactttgtagattttgtttattatcacaatgccacaactttctgctacaactgaaggcattgtcatagttttctttccaagtaaaaatcttagcacttagttaccaggcagcaaaaaaatactgaacttcaagtgaccctaaggaggaactagaagaacctcctagctttcacagtcattagaagttcatcaaggcagttggagctgttcactgggggcagcaacaatgaactgattcattgtcctgaagcaattcctcttatgagcatgtagatgcgatgctaacattcaaactgccatcttaggacgctttgtgcaccttctacttccatccccatctccaaaaactgaaatgctgattcactctgaggatggctatttaagtcaaataattttcagtctaatttttcagttgcattaggaaaagaaaggaaggtaccaacaccaaagctcttggaagaatcgatttggaacagttcaggtttattcctaagggtatctagaggagtgaaagtggtcaggtaatgagtagcaaaggaaaataaattcatacttaaaacactaatttaattaaatcaaagacaagagataaatgtgtataacttacaaaccaacaggagtatgtactttttaaaagtcttgttcttttaaatataaatttagttaggccattgataaaaatgacctgcatttatttatgtatttagactattgatagatgatggtatagtgtgtgtgtgtgtgtgtgtgtgtgtgtgtgtgtgtgttggccaaaaggctgaaaaaccttggaactatagtgttataatttataagtaacatagctcaatgccaatgaaagcccacttagttaaccttgggttggtcccaccatttgccaaatttgatgttaaaacccggattttttgatgcaattacagcaggagcatttaagtgttctttctcttgagctctgtgactgtttctctggaaacctctcattgaattatttggaatggaaatcctaacagggtgggagtttcagaactgagaatcaatgaaaaaggcctcacttccattggggtttagaaattagaaagtatcagatgtttcttggcaatgacatttgggctattgttgcctgtctctcccctgactggcataaaatgtttccacttcgggatgtttgacactgtgtaagtgggagcttggcttagggcttcccatctaagggccaattaacttcaacagcaatcagttcttcagggaaggggttttcagcagagcaaaactctgctctttcacttttaaatactgtctcattttgcttttcattttaccacaatacacacatcaaggtccttccttctgaaaaagccatcagaatattctttctaagctttttacatctatgtgtgggatgagggctgtgaaggaggatgagaagggtttcctggctttattagttccttttagattgtaaaagtgagcttaatagctatatcatttaacatggccacattctggcccaagttacagaaatattataacattgtacaaacagactactgctacaaacaaatctgtttttatgcctcctgcttctttctctcccgtcactgtaattcctgtgattttgaagttggttgccccattaaaaactaataaaacattaatgttttcttgtctttactatgctaaggtttgctttgtagggcaccaaagtagaaatgtactactgattagtggatcttcaactaggaaggtgagaaataacatggaaatgcttaaagcattccaaatgctctctcccctaatttccaacttttgacttactaatgtgtgtgacctagttctgtgacttgtaaggatttattctccaaagatatctttagatgtatgcctgtttcatttgcatccaatactttcatgggaagcctctctatttttgagaagaggaaaaaaattctttgacataaccaccaaaaaagtagaaagttcacttaacgaaactatccttccaaatctgccaaataattcctgcttccttcctaaatcctagctttaaataatgctggacagtgatacagaggccaaatttccctgttgctctctgtacagctggtaggatttgttgttttctctttattcatataggtcctttaggaagtttgtgatacaaaattagaatgctccagtggtttcctccctcttttaaattgctatggatcctaaatatttctgaaattgaaatactacagttatagaatgtttcctgtgtaacttaagcattcacgtaataggaatatgctttagaatttatgaacatctggacttaaaaagatgattaaagattaaaattttcctttttctcaactggggaccctttgaaatctgatttaaatagcatctaaacaggtaaaagaacttagctgaggtttgagaagatggccgtgtttggggaggcaagtctacatcctacggaaagaggagccctaacaagcttcaacataagctctagtccaagagttggtgatggttccagaaagtgatggtggtggtggtgtgcattatgggggttggggaaggcaagtcattgaaaaataagggggcttggaccttggaattccatagctactcatacccttcttggttaaaatgcttgttgcataactggcattcagtagatatgtctcaatctgttcaatgatgttgaatattcacagaattgggaaggatcagtggaaaaagcagtcctgggtagatacttgcttatttaaatgtgtaaacgaagattattgttaaatagccccagtcaggtaatattaatgacttaggaaaattgcaaggaccttaaaaacaacatttcaatttctttataggccaatgatctcagttattaataacagtgaaataaagacacagttcccaacagtaaactgaccagactcgtgacagcgtccctaatcatgagaaaaacttccatttgattttcaactaagagtaaagcaaatgaagtcttgtgacttcttcctctgcacgcatgcgggcatgcgtgcacacacacacacacacacacacacacaagcaattccttggtcatcattcctacaagtgaatagcataatttgaatcaatgggacaaaagccagttgtagtgagattatagtctgatgtcccagaagtagtctgagaacaaatttgaaacaaaaagagcctagcagacaaataaataacaagtcacatgcaggtaccagatgtttatagatggatagtccttataaatttaagatcacatatttgccacatattaaacaggaaagctcccaagaattgaatgcgtacgagccattgacatcaatttattccttcaaataattgttaggcagtataaatgaaggctaatagaccatttacaaatgctgtttgttggcaaccagagccccctggagctgcctgtgtgcacggggacactagcaggcacagttgggctgcggtggaggaggagtttccttgagtctcgtgttctgctttgcagcagtgatggcaggatcagtctccaaactctctgacattttgtcgcagatgatatccacaaggcgctcaaatgtctgcttgacattaatgttgtccttggcacttgtttcaaaaaactcaaacccaagctgttctcctaaatgttgacctcgctcagttgagatgacccgctcgtcttccatgtcacacttgttcccaaccagaataacttgggcattgtcccaagagtatgttttgatttgagttgaccaatcttgtactgcattgaaggattcttcatttgtaatgtcatacattaaaataaagcccatggctccacgataataggctgtggtgatagtcctgtatctttcctggcctgctgtgtcccaaatctgaagcttgattctcttttcatttttgaatacagtttttactttgaaatcgatcccaactgtgctgacgaatgcagatgtaaaggagtcatctgcataacggaatagaaaagatgttttccccacactgctattgccgatgatgagtaatttgaacatgtagtcaaagttctgatcagaggagtctttctggccgtacctggcatcttgggcagaggccatctgcatgggcgcttcgtgtctcattgttggcaaatgtcctttctctctggctaggaccgcactggtctgggcttccggtcaagcgtgcacagtcccggcgctccacgctccacactctgcactcttggggttcgctaaccggctccaacatcagcact

SEQ ID NO: 16722 - RNA, 7120 nt, Homo sapiens
  source 1..7120: mol_type = other RNA
taaatttcacctttctgagaagaaaaacatgacttttcctaatgcacatagtttttcttaggtatctaaattagttgcttaaaagtaaaatgtacacttttatatgacacttaaagaaaattttgagttatagaaggagatgcttttataaaataaatgaacagccattctgtcttgacaataaaatccacaattctaagagataaaattgacacatatttccagatactaaatgtttggttttataagaaaaaagtattttgaagtaggcacagaggggttttacatgacaccaataagatatttactgtataaattgcaccactagacaaatacagctacaagaaaatcatttgaataagtcacacagctatcaaagcatctcacacattcattataattcactctttcatactagtttatatacactgagtgagtcattaaatattgcacttattggcccatgaaccctcaattctgaggtgttgaaaatagaaaacaaatctatttttataacatatttcatgcaacatttaagacatatcagttctacaaacaccattaaattgttgtacatttggacagtctaacggtatcacatcacgtctgacattaacaatatattaacaggaattacaggacagttttcctttagcacgtatcctagggataatgagacaatgcatggaaagccatcatattgatacagcaaacaatacccaaactttacttttacaagaagtatggaaccacttgacagatgtaagtcatgctcacgtccctgaaagggcaggtgtctgaggggctcaggtaccatctgtgtctgtaagaacagcattcacgaacctaagcaatacctagccccaaataacatgaatgcaaaataatttgcctcaagaaataaagccacagccaactctcacttgtccacgatgaaggaaatattaacacaggtgaatgaaatacacaggtaacctcaaacctcatttcagcaagtaatgactgtttgaaactccaccagtaatggttgctgatgggaagtaaatggtgaaatttgagtctcattttctattcttggtcctgtcattccatgaggatagtgttttgaaaaactgcagtaatttaaaagaaagtcagaaagtaaaagagaactgcaaatagaaagttcaatttgtccactagctagatggtctgatcttaacactcgagctctgagtgaggttttaaaatgactcatttctgttatctagaatgcttgcaaaatttatttcccctccactctctctgtttggaggaaattaattacatgcacagactaatcaaacgaaatcagtgtgaagaaccgattttatggaccttataagtaagatgtgagttatagctggaacatagtaaaagctcccttttccctagcactgagaaagcaccatagatggaattttgccttcttaaaaaaaagtatcagtgtttgcctgatacctttgtacaggcgagtgagcgtgtgagtgactgttgagaagggcagcactgtatgtgtaatctaaaagcaaatatttcaatctatcaaagggaaatattatttgaccggagtgtcaagcatttctgtaaatatttttaagaaaaaaattatttgtgaaataccagtaacaataggtagatacattttagataaatcccccaacttggtttttccctgttagggggtactatatttctacaacctagagccctttagatacagtgctgtgcaggggtaaaggcttttttattctggtcataaacttcatcttttacttaatttggcccagtaaattccatgatataaaacaggtttatgtctttaattgactttggtcaaaaattcacctaaaatatgaagaactcccaaaagctggctcaaaggttcagcatatcagaaagacttcaccattttacaggcaaactactaaagcgaaggtaatcaatgcacacaggcagagctgagcagagctgtagaggttgcattttccagggagtgacagaaaggccacatgggtgtagttgctcatgtggcacccggacagcacactaagtgactatacacgcaaaggaacagagttccgggttctagtcatgcaaactgtaattgtgagagaaagggttcttcagacggacaggccagctctgaagtatgccacaccaaaaataactgattgagcattccagtagtactatgaagattattaacaaacacacagtaactttttggtctagaagggttttagttatgacttttttataaataagattcatatcacagtttttcacatgcaggtgttacctacctcagcttggtatagcttggtagtttggatatgcttttaatatagtcccacaaatgccacactgttaactaaaatatcacatagtacatcctcaaccatgcactaagatacatgttggataaagcacatcacaatgaaccactgattatggactaccatgctctaaaattaatgttgcttcatggaagttcagttaatagtggaatgtatttaacttttaaaagagaagaagaaggttgtatatacccgaaagtctatcgtcagcatagatgtatttaaaattgaaagtttaaattggttccttaaaaaataaccagtgtactaaacaaaaggcctataattaatatgaataagatttaagtaggtgaaatatatatatttgtttactgagtgttttgatgtcttgtataatttgggttgtaactttgtagattttgtttattatcacaatgccacaactttctgctacaactgaaggcattgtcatagttttctttccaagtaaaaatcttagcacttagttaccaggcagcaaaaaaatactgaacttcaagtgaccctaaggaggaactagaagaacctcctagctttcacagtcattagaagttcatcaaggcagttggagctgttcactgggggcagcaacaatgaactgattcattgtcctgaagcaattcctcttatgagcatgtagatgcgatgctaacattcaaactgccatcttaggacgctttgtgcaccttctacttccatccccatctccaaaaactgaaatgctgattcactctgaggatggctatttaagtcaaataattttcagtctaatttttcagttgcattaggaaaagaaaggaaggtaccaacaccaaagctcttggaagaatcgatttggaacagttcaggtttattcctaagggtatctagaggagtgaaagtggtcaggtaatgagtagcaaaggaaaataaattcatacttaaaacactaatttaattaaatcaaagacaagagataaatgtgtataacttacaaaccaacaggagtatgtactttttaaaagtcttgttcttttaaatataaatttagttaggccattgataaaaatgacctgcatttatttatgtatttagactattgatagatgatggtatagtgtgtgtgtgtgtgtgtgtgtgtgtgtgtgtgtgtgttggccaaaaggctgaaaaaccttggaactatagtgttataatttataagtaacatagctcaatgccaatgaaagcccacttagttaaccttgggttggtcccaccatttgccaaatttgatgttaaaacccggattttttgatgcaattacagcaggagcatttaagtgttctttctcttgagctctgtgactgtttctctggaaacctctcattgaattatttggaatggaaatcctaacagggtgggagtttcagaactgagaatcaatgaaaaaggcctcacttccattggggtttagaaattagaaagtatcagatgtttcttggcaatgacatttgggctattgttgcctgtctctcccctgactggcataaaatgtttccacttcgggatgtttgacactgtgtaagtgggagcttggcttagggcttcccatctaagggccaattaacttcaacagcaatcagttcttcagggaaggggttttcagcagagcaaaactctgctctttcacttttaaatactgtctcattttgcttttcattttaccacaatacacacatcaaggtccttccttctgaaaaagccatcagaatattctttctaagctttttacatctatgtgtgggatgagggctgtgaaggaggatgagaagggtttcctggctttattagttccttttagattgtaaaagtgagcttaatagctatatcatttaacatggccacattctggcccaagttacagaaatattataacattgtacaaacagactactgctacaaacaaatctgtttttatgcctcctgcttctttctctcccgtcactgtaattcctgtgattttgaagttggttgccccattaaaaactaataaaacattaatgttttcttgtctttactatgctaaggtttgctttgtagggcaccaaagtagaaatgtactactgattagtggatcttcaactaggaaggtgagaaataacatggaaatgcttaaagcattccaaatgctctctcccctaatttccaacttttgacttactaatgtgtgtgacctagttctgtgacttgtaaggatttattctccaaagatatctttagatgtatgcctgtttcatttgcatccaatactttcatgggaagcctctctatttttgagaagaggaaaaaaattctttgacataaccaccaaaaaagtagaaagttcacttaacgaaactatccttccaaatctgccaaataattcctgcttccttcctaaatcctagctttaaataatgctggacagtgatacagaggccaaatttccctgttgctctctgtacagctggtaggatttgttgttttctctttattcatataggtcctttaggaagtttgtgatacaaaattagaatgctccagtggtttcctccctcttttaaattgctatggatcctaaatatttctgaaattgaaatactacagttatagaatgtttcctgtgtaacttaagcattcacgtaataggaatatgctttagaatttatgaacatctggacttaaaaagatgattaaagattaaaattttcctttttctcaactggggaccctttgaaatctgatttaaatagcatctaaacaggtaaaagaacttagctgaggtttgagaagatggccgtgtttggggaggcaagtctacatcctacggaaagaggagccctaacaagcttcaacataagctctagtccaagagttggtgatggttccagaaagtgatggtggtggtggtgtgcattatgggggttggggaaggcaagtcattgaaaaataagggggcttggaccttggaattccatagctactcatacccttcttggttaaaatgcttgttgcataactggcattcagtagatatgtctcaatctgttcaatgatgttgaatattcacagaattgggaaggatcagtggaaaaagcagtcctgggtagatacttgcttatttaaatgtgtaaacgaagattattgttaaatagccccagtcaggtaatattaatgacttaggaaaattgcaaggaccttaaaaacaacatttcaatttctttataggccaatgatctcagttattaataacagtgaaataaagacacagttcccaacagtaaactgaccagactcgtgacagcgtccctaatcatgagaaaaacttccatttgattttcaactaagagtaaagcaaatgaagtcttgtgacttcttcctctgcacgcatgcgggcatgcgtgcacacacacacacacacacacacacacaagcaattccttggtcatcattcctacaagtgaatagcataatttgaatcaatgggacaaaagccagttgtagtgagattatagtctgatgtcccagaagtagtctgagaacaaatttgaaacaaaaagagcctagcagacaaataaataacaagtcacatgcaggtaccagatgtttatagatggatagtccttataaatttaagatcacatatttgccacatattaaacaggaaagctcccaagaattgaatgcgtacgagccattgacatcaatttattccttcaaataattgttaggcagtataaatgaaggctaatagaccatttacaaatgctgtttgttggcaaccagagccccctggagctgcctgtgtgcacggggacactagcaggcacagttgggctgcggtggaggaggagtttccttgagtctcgtgttctgctttgcagcagtgatggcaggatcagtctccaaactctctgacattttgtcgcagatgatatccacaaggcgctcaaatgtctgcttgacattaatgttgtccttggcacttgtttcaaaaaactcaaacccaagctgttctcctaaatgttgacctcgctcagttgagatgacccgctcgtcttccatgtcacacttgttcccaaccagaataacttgggcattgtcccaagagtatgttttgatttgagttgaccaatcttgtactgcattgaaggattcttcatttgtaatgtcatacattaaaataaagcccatggctccacgataataggctgtggtgatagtcctgtatctttcctggcctgctgtgtcccaaatctgaagcttgattctcttttcatttttgaatacagtttttactttgaaatcgatcccaactgtgctgacgaatgcagatgtaaaggagtcatctgcataacggaatagaaaagatgttttccccacactgctattgccgatgatgagtaatttgaacatgtagtcaaagttctgatcagaggagtctttctggccgtacctggcatcttgggcagaggccatctttccatacagctccattacaactcgaggttcagaaattctcaagtgccctcgctacaaaggaggttagggctctacgtaggaagcggggctaaaatgaaaaggcacaacacaatagaaggggtaggggtggcgtctggcggagagaaaaaggagggatgtggagaagacagctgatttagatggagggcttctttcctctggagggaaagcgtggaatccaagctgcagctgcagagaaagggctcagtctcttaggaagt

SEQ ID NO: 16723 - RNA, 5124 nt, Homo sapiens
  source 1..5124: mol_type = other RNA
taaatttcacctttctgagaagagaaggggctcctgcagtagcctaggaaaatcacatttagaatccactcccgggatgtcattctaggctctgctgactacaacagcctgagtgaggaggaaagaggcagcagcagacagcggatgtggagcaagtaccctctggatgtgcagaaggagttcggctatgacagcccccacgacctggattcagactgatggtcttgtgatgtccatgaggttctgccacatgcccttgagggctctgagtccagagttaactgccctgctgacatcctgttaggtttcctagcttaacatgtggaaggaaaagcatatcaagcatatcgggcggcaccatcccaccacagtgaaaacttatgttaggggagtgagtcttttccacttacagtaggacccctttgcctcaatcaaaagtgaccctacagtttgaaagaaaaaaaaacgttgaaaaaaggaaggtttctttagctttagcttcttggcccaggaatttttcctggcattcaggttctgtgctgaaaccacaagggagggggaggttcccatttcattagcagtaagcttctgctgtgccataccaccaggctgcctgcctctaggaaaaccctgttccttttgatagaatctaaaaggggtaccagtgggtcccttgtagcaatacagactggatagtaatggccattagggcagaaagtagtctgagcagtgggagattttagttaacagctatttctgcttccaaactctgataacggttgtgaaattactgactgacttcctttggcagtggggccaagaaacaatatatatgaatgtgatacatgtgtttagtaaaatctagctttgaacatggaagaaagtaattctttgaaaaccttttaaatctgaatatctaaaacagggagcggtagtgaaatagaaggttcagcattgattataaataccaaggacttaaggcaagggaggaaaaacaaagtaccttctgaacttagctttccactgagtaatgtttactcttcacagcacccaccacaaaaacaaactactatcaacaggatcaattttattaacaacttgtatctcttctaagcagactctgtccgtatgcctttccaaaccatagctgccttaactgactgccttggtgtttattctagcgtaacattgtccagtagaactatctgcagtgatgatatgttctgtgtctgcactgtgtagtagtagacacgggtggctgctgagcacttgaaatgtgattagcgcaactgagaaactgagcttttaattttatttcattttaatgtaattagctacacgtggctagtagctgttgcagcggacaccacaggtctaaggaaacaacacagaacattcagctaggggtgtaccctcatagcctgtgagtgtctcttactcactgtcatgggggaaggtgagttacacagggaggtaccttcttgccgcctcttttaggatttcctaagtatctctccttcatcctacctgccatcattctttgactttatgtccattttctaaacctttgcctacacttgctcttatctacatggagttgttcaacctgccgaagtgattaaattctgtgtacacaggccgtatatattgcagctaattaaaacaacaaacatcctaggcatgcacaaaggtataattcaccgttataacaggcagcaacttgtatgtctaatattagacatcttgctttctgtctgtaggcatagaaacaaaggattgaaagccattctcatacagcaaccgggtgaaaaaaacaaaacactgtgctgttacaatgtgctccctgctatttatactcattaagtttccccaatattaaagggctgacaacttaataaactgtactcactgcaaaagggataataagcacaccaggaaaaggatttaaggagacagacaacaaagagctggcagaaattaattccaccatgaagcttgagtgctgtagggatcctctggcttcgctcccaaagagaggatcctgggagaagtctgtatccagcacagaggggaaaaatgctgtcaccatccaaaaatgaaaggaggatgacatggctcactaagcaagtactagggcacctggcatgtgaggtccttgctttccctagaagccactggtggggggcagcaaattcctgggattagctggttatctggtggagaaagctaaagctggggtcagggatctttaaaaggcaagcacattttgcttaaaggattagctccagaggagccctgggatgggtgccagcttagctcagacagaagtcatgttcttagcgttcaggcaagtcagcctttgcataagacaccctgtcgtcgggcaggaatttgccgttacaaatcccaaacccatgacagtaggaatgtcaccccatgcttcacatatgcattatgctctgaacccagggcaactatgaccatgcttccttcaatctttattgagcaaatatatggccaaggttattcccttatctgtgactgggtggagaagaatggtcaggaagggagactgcctcactgttgaccaattccaaaacctaaggataagcccatggggtatgtcaagctagcaggttcttctcggcccaggatgacagtgtctgggggcatcacaaaacagttgtacaatccaatgcagccgtcctgctcatacagtaagatccattaggccagagcaggcctaacttgggtggagagcccagcctgagcaccagaattagttgcttccacttgtgcagcctgctgaagagccggactcaggttgaagcagctttcctcccagtcttcactgatctccacagggagaaaacagaagtccccacaagtaccaagctcttcctgagactgcagccaccacacctcggggaaggggaggctggcaggagaggagtacactgtcccggtgacccacaccaaggtggctccaagtgtaaacaaagccaataagagtgagcactggccctgagccccactatatgattgggtcaaaaggctcctttaattcaggagagttgggcccacagagtcttgttatcaggattttgctggttggcctgccttccaggcctcagaaagccacctctgacctctagtcagttttcctctcatcctttttttcttcggctacatcaagctcagtcaggacacaaaagcaaagctgctgggtgcctctggtgatagcagccaggacattccgaataaacaatggcctccgggactctggcaggtaaacacccatgaagtagaaagggactccagaaagggcaatcccgatgccaatgagggaattaatggtgtcagtgaagaggggcactatcaccagaaacacggagcatatgcagaacacgatggggaaaaacacgctcagcttgagaggccggggccgcttgggctccttccagcggaggtagagctgtccaacaacagacaggcccacgaagaaccagtagctgaagctgaagtagttgataagctggaaaacatcctccacgatgaggtagatgagtgccatggtgcaattgaacagtaaagcagggataggtgtaaaacgctcaatgtggatcatggacagaaggtccggtaggtggccctcccgggagcccacgaagaacaaccttgatgaagcaaagatggatgcattgaggcccccaaagcaggacagggcaacagcaatggggatggtccagctgaacatgccaaacgtctggtcagcaaatgtcacagccacagcatcactgctaaggacatctgaaatgttcagcactgtgtaataggccacattggtcaggatgtagatgagcgtcacaattggcatagaaatcccaatggccaagggcaaatttctttctgggtttttgatttcttctgttacaaaattaagggtgtcccaacctgagtaagagaagagggcagagtagagggcaagagagaggtttcccatgtcccaggaggaaccctcaaaggcgtcctgaaagtgctcagagtgtccctggcacagtttaacaaggcccatgacaatgatggcaatgagcgctacgaccttggcgtaagtgaacgtgtcctgcacacgtgtgccccacttgacataggcacagttcacaaatgtcagcagacatatgcaagcagcagccaggagacggcaggccaggtatgggggatcacagctggggaaggacggctggatgatgtagttggcaaaggtgatggcgatgatggcctgaccggtgggctcaacaactagcagtgagacccacaggcggatgaaggcaatgaagcccccaaaggcctctagaatataagcgtagctggctcccgacttggtgatggtggtccccagctctgcataacaaagggcacccacaacagagaagagcccaccaatggcccacacaatcagtgacatcccataggaggcagtgtgtaccagcacacccttgggtgagacaaagatccctgagccgatcatgttgcccaccaccaggctgaccccattcagcagggagatctccttcttcagctgcatagtttcggaggacctttgaggtggcgagctgacatcttcttccacctgggactggctggtgttagggacaagatggtaggtgggtgtgggcctcccaggctccctggcttccatgacaaacggttcctgcacacctgtgtttgctgtggcctgtaatccccactcaggaggctgaggcaggagaatcgcttgaaccagggagtcggaggttgcagtgagccaagatcacgccactgcctgtcaagaaatacgcgaacatcacactttcataagccacctcctcataaatgggtccagtactgagaaggaaatgaagtcccctgcagcaaggcctaattccacttgtctgcctcggccacataaactccgcagcgcctctcgcgcggccccgatcggccagccccgcgctgtttctgggccgcatcccgctcccgacggcggcagcgaagacccacagggttcggctcccacagaacgcggcccagccccggccccgctcccggcgcgcccgcccatggcccagcccgttacctcccagt

SEQ ID NO: 16724 - RNA, 4978 nt, Homo sapiens
  source 1..4978: mol_type = other RNA
taaatttcacctttctgagaagagaaggggctcctgcagtagcctaggaaaatcacatttagaatccactcccgggatgtcattctaggctctgctgactacaacagcctgagtgaggaggaaagaggcagcagcagacagcggatgtggagcaagtaccctctggatgtgcagaaggagttcggctatgacagcccccacgacctggattcagactgatggtcttgtgatgtccatgaggttctgccacatgcccttgagggctctgagtccagagttaactgccctgctgacatcctgttaggtttcctagcttaacatgtggaaggaaaagcatatcaagcatatcgggcggcaccatcccaccacagtgaaaacttatgttaggggagtgagtcttttccacttacagtaggacccctttgcctcaatcaaaagtgaccctacagtttgaaagaaaaaaaaacgttgaaaaaaggaaggtttctttagctttagcttcttggcccaggaatttttcctggcattcaggttctgtgctgaaaccacaagggagggggaggttcccatttcattagcagtaagcttctgctgtgccataccaccaggctgcctgcctctaggaaaaccctgttccttttgatagaatctaaaaggggtaccagtgggtcccttgtagcaatacagactggatagtaatggccattagggcagaaagtagtctgagcagtgggagattttagttaacagctatttctgcttccaaactctgataacggttgtgaaattactgactgacttcctttggcagtggggccaagaaacaatatatatgaatgtgatacatgtgtttagtaaaatctagctttgaacatggaagaaagtaattctttgaaaaccttttaaatctgaatatctaaaacagggagcggtagtgaaatagaaggttcagcattgattataaataccaaggacttaaggcaagggaggaaaaacaaagtaccttctgaacttagctttccactgagtaatgtttactcttcacagcacccaccacaaaaacaaactactatcaacaggatcaattttattaacaacttgtatctcttctaagcagactctgtccgtatgcctttccaaaccatagctgccttaactgactgccttggtgtttattctagcgtaacattgtccagtagaactatctgcagtgatgatatgttctgtgtctgcactgtgtagtagtagacacgggtggctgctgagcacttgaaatgtgattagcgcaactgagaaactgagcttttaattttatttcattttaatgtaattagctacacgtggctagtagctgttgcagcggacaccacaggtctaaggaaacaacacagaacattcagctaggggtgtaccctcatagcctgtgagtgtctcttactcactgtcatgggggaaggtgagttacacagggaggtaccttcttgccgcctcttttaggatttcctaagtatctctccttcatcctacctgccatcattctttgactttatgtccattttctaaacctttgcctacacttgctcttatctacatggagttgttcaacctgccgaagtgattaaattctgtgtacacaggccgtatatattgcagctaattaaaacaacaaacatcctaggcatgcacaaaggtataattcaccgttataacaggcagcaacttgtatgtctaatattagacatcttgctttctgtctgtaggcatagaaacaaaggattgaaagccattctcatacagcaaccgggtgaaaaaaacaaaacactgtgctgttacaatgtgctccctgctatttatactcattaagtttccccaatattaaagggctgacaacttaataaactgtactcactgcaaaagggataataagcacaccaggaaaaggatttaaggagacagacaacaaagagctggcagaaattaattccaccatgaagcttgagtgctgtagggatcctctggcttcgctcccaaagagaggatcctgggagaagtctgtatccagcacagaggggaaaaatgctgtcaccatccaaaaatgaaaggaggatgacatggctcactaagcaagtactagggcacctggcatgtgaggtccttgctttccctagaagccactggtggggggcagcaaattcctgggattagctggttatctggtggagaaagctaaagctggggtcagggatctttaaaaggcaagcacattttgcttaaaggattagctccagaggagccctgggatgggtgccagcttagctcagacagaagtcatgttcttagcgttcaggcaagtcagcctttgcataagacaccctgtcgtcgggcaggaatttgccgttacaaatcccaaacccatgacagtaggaatgtcaccccatgcttcacatatgcattatgctctgaacccagggcaactatgaccatgcttccttcaatctttattgagcaaatatatggccaaggttattcccttatctgtgactgggtggagaagaatggtcaggaagggagactgcctcactgttgaccaattccaaaacctaaggataagcccatggggtatgtcaagctagcaggttcttctcggcccaggatgacagtgtctgggggcatcacaaaacagttgtacaatccaatgcagccgtcctgctcatacagtaagatccattaggccagagcaggcctaacttgggtggagagcccagcctgagcaccagaattagttgcttccacttgtgcagcctgctgaagagccggactcaggttgaagcagctttcctcccagtcttcactgatctccacagggagaaaacagaagtccccacaagtaccaagctcttcctgagactgcagccaccacacctcggggaaggggaggctggcaggagaggagtacactgtcccggtgacccacaccaaggtggctccaagtgtaaacaaagccaataagagtgagcactggccctgagccccactatatgattgggtcaaaaggctcctttaattcaggagagttgggcccacagagtcttgttatcaggattttgctggttggcctgccttccaggcctcagaaagccacctctgacctctagtcagttttcctctcatcctttttttcttcggctacatcaagctcagtcaggacacaaaagcaaagctgctgggtgcctctggtgatagcagccaggacattccgaataaacaatggcctccgggactctggcaggtaaacacccatgaagtagaaagggactccagaaagggcaatcccgatgccaatgagggaattaatggtgtcagtgaagaggggcactatcaccagaaacacggagcatatgcagaacacgatggggaaaaacacgctcagcttgagaggccggggccgcttgggctccttccagcggaggtagagctgtccaacaacagacaggcccacgaagaaccagtagctgaagctgaagtagttgataagctggaaaacatcctccacgatgaggtagatgagtgccatggtgcaattgaacagtaaagcagggataggtgtaaaacgctcaatgtggatcatggacagaaggtccggtaggtggccctcccgggagcccacgaagaacaaccttgatgaagcaaagatggatgcattgaggcccccaaagcaggacagggcaacagcaatggggatggtccagctgaacatgccaaacgtctggtcagcaaatgtcacagccacagcatcactgctaaggacatctgaaatgttcagcactgtgtaataggccacattggtcaggatgtagatgagcgtcacaattggcatagaaatcccaatggccaagggcaaatttctttctgggtttttgatttcttctgttacaaaattaagggtgtcccaacctgagtaagagaagagggcagagtagagggcaagagagaggtttcccatgtcccaggaggaaccctcaaaggcgtcctgaaagtgctcagagtgtccctggcacagtttaacaaggcccatgacaatgatggcaatgagcgctacgaccttggcgtaagtgaacgtgtcctgcacacgtgtgccccacttgacataggcacagttcacaaatgtcagcagacatatgcaagcagcagccaggagacggcaggccaggtatgggggatcacagctggggaaggacggctggatgatgtagttggcaaaggtgatggcgatgatggcctgaccggtgggctcaacaactagcagtgagacccacaggcggatgaaggcaatgaagcccccaaaggcctctagaatataagcgtagctggctcccgacttggtgatggtggtccccagctctgcataacaaagggcacccacaacagagaagagcccaccaatggcccacacaatcagtgacatcccataggaggcagtgtgtaccagcacacccttgggtgagacaaagatccctgagccgatcatgttgcccaccaccaggctgaccccattcagcagggagatctccttcttcagctgcatagtttcggaggacctttgaggtggcgagctgacatcttcttccacctgggactggctggtgttagggacaagatggtaggtgggtgtgggcctcccaggctccctggcttccatgacaaacggttcctgcacacctgtgtttgctgtggcctgtaatccccactcaggaggctgaggcaggagaatcgcttgaaccagggagtcggaggttgcagtgagccaagatcacgccactgcctgtcaagaaatacgcgaacatcacactttcataagccacctcctcataaatgggtccagtactgagaaggaaatgaagtcccctgcagcaaggcctaattccacttgtctgcctcggccacataaactctcccagtggcccggcgccgccaggat

SEQ ID NO: 16725 - RNA, 4925 nt, Homo sapiens
  source 1..4925: mol_type = other RNA
taaatttcacctttctgagaagagaaggggctcctgcagtagcctaggaaaatcacatttagaatccactcccgggatgtcattctaggctctgctgactacaacagcctgagtgaggaggaaagaggcagcagcagacagcggatgtggagcaagtaccctctggatgtgcagaaggagttcggctatgacagcccccacgacctggattcagactgatggtcttgtgatgtccatgaggttctgccacatgcccttgagggctctgagtccagagttaactgccctgctgacatcctgttaggtttcctagcttaacatgtggaaggaaaagcatatcaagcatatcgggcggcaccatcccaccacagtgaaaacttatgttaggggagtgagtcttttccacttacagtaggacccctttgcctcaatcaaaagtgaccctacagtttgaaagaaaaaaaaacgttgaaaaaaggaaggtttctttagctttagcttcttggcccaggaatttttcctggcattcaggttctgtgctgaaaccacaagggagggggaggttcccatttcattagcagtaagcttctgctgtgccataccaccaggctgcctgcctctaggaaaaccctgttccttttgatagaatctaaaaggggtaccagtgggtcccttgtagcaatacagactggatagtaatggccattagggcagaaagtagtctgagcagtgggagattttagttaacagctatttctgcttccaaactctgataacggttgtgaaattactgactgacttcctttggcagtggggccaagaaacaatatatatgaatgtgatacatgtgtttagtaaaatctagctttgaacatggaagaaagtaattctttgaaaaccttttaaatctgaatatctaaaacagggagcggtagtgaaatagaaggttcagcattgattataaataccaaggacttaaggcaagggaggaaaaacaaagtaccttctgaacttagctttccactgagtaatgtttactcttcacagcacccaccacaaaaacaaactactatcaacaggatcaattttattaacaacttgtatctcttctaagcagactctgtccgtatgcctttccaaaccatagctgccttaactgactgccttggtgtttattctagcgtaacattgtccagtagaactatctgcagtgatgatatgttctgtgtctgcactgtgtagtagtagacacgggtggctgctgagcacttgaaatgtgattagcgcaactgagaaactgagcttttaattttatttcattttaatgtaattagctacacgtggctagtagctgttgcagcggacaccacaggtctaaggaaacaacacagaacattcagctaggggtgtaccctcatagcctgtgagtgtctcttactcactgtcatgggggaaggtgagttacacagggaggtaccttcttgccgcctcttttaggatttcctaagtatctctccttcatcctacctgccatcattctttgactttatgtccattttctaaacctttgcctacacttgctcttatctacatggagttgttcaacctgccgaagtgattaaattctgtgtacacaggccgtatatattgcagctaattaaaacaacaaacatcctaggcatgcacaaaggtataattcaccgttataacaggcagcaacttgtatgtctaatattagacatcttgctttctgtctgtaggcatagaaacaaaggattgaaagccattctcatacagcaaccgggtgaaaaaaacaaaacactgtgctgttacaatgtgctccctgctatttatactcattaagtttccccaatattaaagggctgacaacttaataaactgtactcactgcaaaagggataataagcacaccaggaaaaggatttaaggagacagacaacaaagagctggcagaaattaattccaccatgaagcttgagtgctgtagggatcctctggcttcgctcccaaagagaggatcctgggagaagtctgtatccagcacagaggggaaaaatgctgtcaccatccaaaaatgaaaggaggatgacatggctcactaagcaagtactagggcacctggcatgtgaggtccttgctttccctagaagccactggtggggggcagcaaattcctgggattagctggttatctggtggagaaagctaaagctggggtcagggatctttaaaaggcaagcacattttgcttaaaggattagctccagaggagccctgggatgggtgccagcttagctcagacagaagtcatgttcttagcgttcaggcaagtcagcctttgcataagacaccctgtcgtcgggcaggaatttgccgttacaaatcccaaacccatgacagtaggaatgtcaccccatgcttcacatatgcattatgctctgaacccagggcaactatgaccatgcttccttcaatctttattgagcaaatatatggccaaggttattcccttatctgtgactgggtggagaagaatggtcaggaagggagactgcctcactgttgaccaattccaaaacctaaggataagcccatggggtatgtcaagctagcaggttcttctcggcccaggatgacagtgtctgggggcatcacaaaacagttgtacaatccaatgcagccgtcctgctcatacagtaagatccattaggccagagcaggcctaacttgggtggagagcccagcctgagcaccagaattagttgcttccacttgtgcagcctgctgaagagccggactcaggttgaagcagctttcctcccagtcttcactgatctccacagggagaaaacagaagtccccacaagtaccaagctcttcctgagactgcagccaccacacctcggggaaggggaggctggcaggagaggagtacactgtcccggtgacccacaccaaggtggctccaagtgtaaacaaagccaataagagtgagcactggccctgagccccactatatgattgggtcaaaaggctcctttaattcaggagagttgggcccacagagtcttgttatcaggattttgctggttggcctgccttccaggcctcagaaagccacctctgacctctagtcagttttcctctcatcctttttttcttcggctacatcaagctcagtcaggacacaaaagcaaagctgctgggtgcctctggtgatagcagccaggacattccgaataaacaatggcctccgggactctggcaggtaaacacccatgaagtagaaagggactccagaaagggcaatcccgatgccaatgagggaattaatggtgtcagtgaagaggggcactatcaccagaaacacggagcatatgcagaacacgatggggaaaaacacgctcagcttgagaggccggggccgcttgggctccttccagcggaggtagagctgtccaacaacagacaggcccacgaagaaccagtagctgaagctgaagtagttgataagctggaaaacatcctccacgatgaggtagatgagtgccatggtgcaattgaacagtaaagcagggataggtgtaaaacgctcaatgtggatcatggacagaaggtccggtaggtggccctcccgggagcccacgaagaacaaccttgatgaagcaaagatggatgcattgaggcccccaaagcaggacagggcaacagcaatggggatggtccagctgaacatgccaaacgtctggtcagcaaatgtcacagccacagcatcactgctaaggacatctgaaatgttcagcactgtgtaataggccacattggtcaggatgtagatgagcgtcacaattggcatagaaatcccaatggccaagggcaaatttctttctgggtttttgatttcttctgttacaaaattaagggtgtcccaacctgagtaagagaagagggcagagtagagggcaagagagaggtttcccatgtcccaggaggaaccctcaaaggcgtcctgaaagtgctcagagtgtccctggcacagtttaacaaggcccatgacaatgatggcaatgagcgctacgaccttggcgtaagtgaacgtgtcctgcacacgtgtgccccacttgacataggcacagttcacaaatgtcagcagacatatgcaagcagcagccaggagacggcaggccaggtatgggggatcacagctggggaaggacggctggatgatgtagttggcaaaggtgatggcgatgatggcctgaccggtgggctcaacaactagcagtgagacccacaggcggatgaaggcaatgaagcccccaaaggcctctagaatataagcgtagctggctcccgacttggtgatggtggtccccagctctgcataacaaagggcacccacaacagagaagagcccaccaatggcccacacaatcagtgacatcccataggaggcagtgtgtaccagcacacccttgggtgagacaaagatccctgagccgatcatgttgcccaccaccaggctgaccccattcagcagggagatctccttcttcagctgcatagtttcggaggacctttgaggtggcgagctgacatcttcttccacctgggactggctggtgttagggacaagatggtaggtgggtgtgggcctcccaggctccctggcttccatgacaaacggttcctgcacacctgtgtttgctgtggcctgtcaagaaatacgcgaacatcacactttcataagccacctcctcataaatgggtccagtactgagaaggaaatgaagtcccctgcagcaaggcctaattccacttgtctgcctcggccacataaactctcccagtggcccggcgccgccaggatgctcggtcgcgccgccgccgccgcggcagctcag

SEQ ID NO: 16726 - RNA, 5816 nt, Homo sapiens
  source 1..5816: mol_type = other RNA
taaatttcacctttctgagaagagaaggggctcctgcagtagcctaggaaaatcacatttagaatccactcccgggatgtcattctaggctctgctgactacaacagcctgagtgaggaggaaagaggcagcagcagacagcggatgtggagcaagtaccctctggatgtgcagaaggagttcggctatgacagcccccacgacctggattcagactgatggtcttgtgatgtccatgaggttctgccacatgcccttgagggctctgagtccagagttaactgccctgctgacatcctgttaggtttcctagcttaacatgtggaaggaaaagcatatcaagcatatcgggcggcaccatcccaccacagtgaaaacttatgttaggggagtgagtcttttccacttacagtaggacccctttgcctcaatcaaaagtgaccctacagtttgaaagaaaaaaaaacgttgaaaaaaggaaggtttctttagctttagcttcttggcccaggaatttttcctggcattcaggttctgtgctgaaaccacaagggagggggaggttcccatttcattagcagtaagcttctgctgtgccataccaccaggctgcctgcctctaggaaaaccctgttccttttgatagaatctaaaaggggtaccagtgggtcccttgtagcaatacagactggatagtaatggccattagggcagaaagtagtctgagcagtgggagattttagttaacagctatttctgcttccaaactctgataacggttgtgaaattactgactgacttcctttggcagtggggccaagaaacaatatatatgaatgtgatacatgtgtttagtaaaatctagctttgaacatggaagaaagtaattctttgaaaaccttttaaatctgaatatctaaaacagggagcggtagtgaaatagaaggttcagcattgattataaataccaaggacttaaggcaagggaggaaaaacaaagtaccttctgaacttagctttccactgagtaatgtttactcttcacagcacccaccacaaaaacaaactactatcaacaggatcaattttattaacaacttgtatctcttctaagcagactctgtccgtatgcctttccaaaccatagctgccttaactgactgccttggtgtttattctagcgtaacattgtccagtagaactatctgcagtgatgatatgttctgtgtctgcactgtgtagtagtagacacgggtggctgctgagcacttgaaatgtgattagcgcaactgagaaactgagcttttaattttatttcattttaatgtaattagctacacgtggctagtagctgttgcagcggacaccacaggtctaaggaaacaacacagaacattcagctaggggtgtaccctcatagcctgtgagtgtctcttactcactgtcatgggggaaggtgagttacacagggaggtaccttcttgccgcctcttttaggatttcctaagtatctctccttcatcctacctgccatcattctttgactttatgtccattttctaaacctttgcctacacttgctcttatctacatggagttgttcaacctgccgaagtgattaaattctgtgtacacaggccgtatatattgcagctaattaaaacaacaaacatcctaggcatgcacaaaggtataattcaccgttataacaggcagcaacttgtatgtctaatattagacatcttgctttctgtctgtaggcatagaaacaaaggattgaaagccattctcatacagcaaccgggtgaaaaaaacaaaacactgtgctgttacaatgtgctccctgctatttatactcattaagtttccccaatattaaagggctgacaacttaataaactgtactcactgcaaaagggataataagcacaccaggaaaaggatttaaggagacagacaacaaagagctggcagaaattaattccaccatgaagcttgagtgctgtagggatcctctggcttcgctcccaaagagaggatcctgggagaagtctgtatccagcacagaggggaaaaatgctgtcaccatccaaaaatgaaaggaggatgacatggctcactaagcaagtactagggcacctggcatgtgaggtccttgctttccctagaagccactggtggggggcagcaaattcctgggattagctggttatctggtggagaaagctaaagctggggtcagggatctttaaaaggcaagcacattttgcttaaaggattagctccagaggagccctgggatgggtgccagcttagctcagacagaagtcatgttcttagcgttcaggcaagtcagcctttgcataagacaccctgtcgtcgggcaggaatttgccgttacaaatcccaaacccatgacagtaggaatgtcaccccatgcttcacatatgcattatgctctgaacccagggcaactatgaccatgcttccttcaatctttattgagcaaatatatggccaaggttattcccttatctgtgactgggtggagaagaatggtcaggaagggagactgcctcactgttgaccaattccaaaacctaaggataagcccatggggtatgtcaagctagcaggttcttctcggcccaggatgacagtgtctgggggcatcacaaaacagttgtacaatccaatgcagccgtcctgctcatacagtaagatccattaggccagagcaggcctaacttgggtggagagcccagcctgagcaccagaattagttgcttccacttgtgcagcctgctgaagagccggactcaggttgaagcagctttcctcccagtcttcactgatctccacagggagaaaacagaagtccccacaagtaccaagctcttcctgagactgcagccaccacacctcggggaaggggaggctggcaggagaggagtacactgtcccggtgacccacaccaaggtggctccaagtgtaaacaaagcctggtgccagggacagaagaggatgcagcctgatgtgaggttttcagaaaagtgaaatgacctagcaccaggttgggattgcttgggtctgcacagcagtccctcacactgcccttacagagaggaacaggttatttgatgacttgggcccatgagatgttctccaagccattgacagctgagagaattcaggtgatccacctgaatatcagaagtttcagccctcttagagttcgtaacagaaacccagagatttactgtcagctagaacaaagatgtaaggtctcaagtaaaataaaggattgtccttcaaaacagcaatattaacagacttctgactcaggaatttgttcatctgtccttgctggacctgagccaagtgcttgtaacgtgatctatgatctatctgtatgctaaagtgtaacaggtacgtgagtaaaaaaatctttaaggttcattgttgcaggtaagactcaatagaaattgtgctaaacagcataaaacctgtggtcagagtctgacccaataccacagacatttctgagcccaaagggactcagttttgggtactttgatttttaaatacaatcagcctattgcatcctgtagatgaagagacacgcatgcttcgttagaactggtgttctggactaaatatcaataaataagggaatataactctctccccagggaagaattttgagccagaggaagaaatggtagcatttcaggcctttaaagtcaggtgttgtacctggtcagagaaaaacttcccataaagcagcccctctatagggactcctagttcaaataccaaattcagaagccaccagccctatcaacctagcattccctcttccccactgcactttaccaagtaaatatctgtaagagctgcatctacctatcaggagtaaaactaaatgaccattccccccgttccccaatcttccccccaccctctgaagcccccaccttgaggttggcccagatcctgagtctcctatagcttaccaataagagtgagcactggccctgagccccactatatgattgggtcaaaaggctcctttaattcaggagagttgggcccacagagtcttgttatcaggattttgctggttggcctgccttccaggcctcagaaagccacctctgacctctagtcagttttcctctcatcctttttttcttcggctacatcaagctcagtcaggacacaaaagcaaagctgctgggtgcctctggtgatagcagccaggacattccgaataaacaatggcctccgggactctggcaggtaaacacccatgaagtagaaagggactccagaaagggcaatcccgatgccaatgagggaattaatggtgtcagtgaagaggggcactatcaccagaaacacggagcatatgcagaacacgatggggaaaaacacgctcagcttgagaggccggggccgcttgggctccttccagcggaggtagagctgtccaacaacagacaggcccacgaagaaccagtagctgaagctgaagtagttgataagctggaaaacatcctccacgatgaggtagatgagtgccatggtgcaattgaacagtaaagcagggataggtgtaaaacgctcaatgtggatcatggacagaaggtccggtaggtggccctcccgggagcccacgaagaacaaccttgatgaagcaaagatggatgcattgaggcccccaaagcaggacagggcaacagcaatggggatggtccagctgaacatgccaaacgtctggtcagcaaatgtcacagccacagcatcactgctaaggacatctgaaatgttcagcactgtgtaataggccacattggtcaggatgtagatgagcgtcacaattggcatagaaatcccaatggccaagggcaaatttctttctgggtttttgatttcttctgttacaaaattaagggtgtcccaacctgagtaagagaagagggcagagtagagggcaagagagaggtttcccatgtcccaggaggaaccctcaaaggcgtcctgaaagtgctcagagtgtccctggcacagtttaacaaggcccatgacaatgatggcaatgagcgctacgaccttggcgtaagtgaacgtgtcctgcacacgtgtgccccacttgacataggcacagttcacaaatgtcagcagacatatgcaagcagcagccaggagacggcaggccaggtatgggggatcacagctggggaaggacggctggatgatgtagttggcaaaggtgatggcgatgatggcctgaccggtgggctcaacaactagcagtgagacccacaggcggatgaaggcaatgaagcccccaaaggcctctagaatataagcgtagctggctcccgacttggtgatggtggtccccagctctgcataacaaagggcacccacaacagagaagagcccaccaatggcccacacaatcagtgacatcccataggaggcagtgtgtaccagcacacccttgggtgagacaaagatccctgagccgatcatgttgcccaccaccaggctgaccccattcagcagggagatctccttcttcagctgcatagtttcggaggacctttgaggtggcgagctgacatcttcttccacctgggactggctggtgttagggacaagatggtaggtgggtgtgggcctcccaggctccctggcttccatgacaaacggttcctgcacacctgtgtttgctgtggcctcccagtggcccggcgccgccaggatgctcggtcgcgccgccgccgccgcggcagctcaggccccg

SEQ ID NO: 16727 - RNA, 5988 nt, Homo sapiens
  source 1..5988: mol_type = other RNA
taaatttcacctttctgagaagagaaggggctcctgcagtagcctaggaaaatcacatttagaatccactcccgggatgtcattctaggctctgctgactacaacagcctgagtgaggaggaaagaggcagcagcagacagcggatgtggagcaagtaccctctggatgtgcagaaggagttcggctatgacagcccccacgacctggattcagactgatggtcttgtgatgtccatgaggttctgccacatgcccttgagggctctgagtccagagttaactgccctgctgacatcctgttaggtttcctagcttaacatgtggaaggaaaagcatatcaagcatatcgggcggcaccatcccaccacagtgaaaacttatgttaggggagtgagtcttttccacttacagtaggacccctttgcctcaatcaaaagtgaccctacagtttgaaagaaaaaaaaacgttgaaaaaaggaaggtttctttagctttagcttcttggcccaggaatttttcctggcattcaggttctgtgctgaaaccacaagggagggggaggttcccatttcattagcagtaagcttctgctgtgccataccaccaggctgcctgcctctaggaaaaccctgttccttttgatagaatctaaaaggggtaccagtgggtcccttgtagcaatacagactggatagtaatggccattagggcagaaagtagtctgagcagtgggagattttagttaacagctatttctgcttccaaactctgataacggttgtgaaattactgactgacttcctttggcagtggggccaagaaacaatatatatgaatgtgatacatgtgtttagtaaaatctagctttgaacatggaagaaagtaattctttgaaaaccttttaaatctgaatatctaaaacagggagcggtagtgaaatagaaggttcagcattgattataaataccaaggacttaaggcaagggaggaaaaacaaagtaccttctgaacttagctttccactgagtaatgtttactcttcacagcacccaccacaaaaacaaactactatcaacaggatcaattttattaacaacttgtatctcttctaagcagactctgtccgtatgcctttccaaaccatagctgccttaactgactgccttggtgtttattctagcgtaacattgtccagtagaactatctgcagtgatgatatgttctgtgtctgcactgtgtagtagtagacacgggtggctgctgagcacttgaaatgtgattagcgcaactgagaaactgagcttttaattttatttcattttaatgtaattagctacacgtggctagtagctgttgcagcggacaccacaggtctaaggaaacaacacagaacattcagctaggggtgtaccctcatagcctgtgagtgtctcttactcactgtcatgggggaaggtgagttacacagggaggtaccttcttgccgcctcttttaggatttcctaagtatctctccttcatcctacctgccatcattctttgactttatgtccattttctaaacctttgcctacacttgctcttatctacatggagttgttcaacctgccgaagtgattaaattctgtgtacacaggccgtatatattgcagctaattaaaacaacaaacatcctaggcatgcacaaaggtataattcaccgttataacaggcagcaacttgtatgtctaatattagacatcttgctttctgtctgtaggcatagaaacaaaggattgaaagccattctcatacagcaaccgggtgaaaaaaacaaaacactgtgctgttacaatgtgctccctgctatttatactcattaagtttccccaatattaaagggctgacaacttaataaactgtactcactgcaaaagggataataagcacaccaggaaaaggatttaaggagacagacaacaaagagctggcagaaattaattccaccatgaagcttgagtgctgtagggatcctctggcttcgctcccaaagagaggatcctgggagaagtctgtatccagcacagaggggaaaaatgctgtcaccatccaaaaatgaaaggaggatgacatggctcactaagcaagtactagggcacctggcatgtgaggtccttgctttccctagaagccactggtggggggcagcaaattcctgggattagctggttatctggtggagaaagctaaagctggggtcagggatctttaaaaggcaagcacattttgcttaaaggattagctccagaggagccctgggatgggtgccagcttagctcagacagaagtcatgttcttagcgttcaggcaagtcagcctttgcataagacaccctgtcgtcgggcaggaatttgccgttacaaatcccaaacccatgacagtaggaatgtcaccccatgcttcacatatgcattatgctctgaacccagggcaactatgaccatgcttccttcaatctttattgagcaaatatatggccaaggttattcccttatctgtgactgggtggagaagaatggtcaggaagggagactgcctcactgttgaccaattccaaaacctaaggataagcccatggggtatgtcaagctagcaggttcttctcggcccaggatgacagtgtctgggggcatcacaaaacagttgtacaatccaatgcagccgtcctgctcatacagtaagatccattaggccagagcaggcctaacttgggtggagagcccagcctgagcaccagaattagttgcttccacttgtgcagcctgctgaagagccggactcaggttgaagcagctttcctcccagtcttcactgatctccacagggagaaaacagaagtccccacaagtaccaagctcttcctgagactgcagccaccacacctcggggaaggggaggctggcaggagaggagtacactgtcccggtgacccacaccaaggtggctccaagtgtaaacaaagcctggtgccagggacagaagaggatgcagcctgatgtgaggttttcagaaaagtgaaatgacctagcaccaggttgggattgcttgggtctgcacagcagtccctcacactgcccttacagagaggaacaggttatttgatgacttgggcccatgagatgttctccaagccattgacagctgagagaattcaggtgatccacctgaatatcagaagtttcagccctcttagagttcgtaacagaaacccagagatttactgtcagctagaacaaagatgtaaggtctcaagtaaaataaaggattgtccttcaaaacagcaatattaacagacttctgactcaggaatttgttcatctgtccttgctggacctgagccaagtgcttgtaacgtgatctatgatctatctgtatgctaaagtgtaacaggtacgtgagtaaaaaaatctttaaggttcattgttgcaggtaagactcaatagaaattgtgctaaacagcataaaacctgtggtcagagtctgacccaataccacagacatttctgagcccaaagggactcagttttgggtactttgatttttaaatacaatcagcctattgcatcctgtagatgaagagacacgcatgcttcgttagaactggtgttctggactaaatatcaataaataagggaatataactctctccccagggaagaattttgagccagaggaagaaatggtagcatttcaggcctttaaagtcaggtgttgtacctggtcagagaaaaacttcccataaagcagcccctctatagggactcctagttcaaataccaaattcagaagccaccagccctatcaacctagcattccctcttccccactgcactttaccaagtaaatatctgtaagagctgcatctacctatcaggagtaaaactaaatgaccattccccccgttccccaatcttccccccaccctctgaagcccccaccttgaggttggcccagatcctgagtctcctatagcttaccaataagagtgagcactggccctgagccccactatatgattgggtcaaaaggctcctttaattcaggagagttgggcccacagagtcttgttatcaggattttgctggttggcctgccttccaggcctcagaaagccacctctgacctctagtcagttttcctctcatcctttttttcttcggctacatcaagctcagtcaggacacaaaagcaaagctgctgggtgcctctggtgatagcagccaggacattccgaataaacaatggcctccgggactctggcaggtaaacacccatgaagtagaaagggactccagaaagggcaatcccgatgccaatgagggaattaatggtgtcagtgaagaggggcactatcaccagaaacacggagcatatgcagaacacgatggggaaaaacacgctcagcttgagaggccggggccgcttgggctccttccagcggaggtagagctgtccaacaacagacaggcccacgaagaaccagtagctgaagctgaagtagttgataagctggaaaacatcctccacgatgaggtagatgagtgccatggtgcaattgaacagtaaagcagggataggtgtaaaacgctcaatgtggatcatggacagaaggtccggtaggtggccctcccgggagcccacgaagaacaaccttgatgaagcaaagatggatgcattgaggcccccaaagcaggacagggcaacagcaatggggatggtccagctgaacatgccaaacgtctggtcagcaaatgtcacagccacagcatcactgctaaggacatctgaaatgttcagcactgtgtaataggccacattggtcaggatgtagatgagcgtcacaattggcatagaaatcccaatggccaagggcaaatttctttctgggtttttgatttcttctgttacaaaattaagggtgtcccaacctgagtaagagaagagggcagagtagagggcaagagagaggtttcccatgtcccaggaggaaccctcaaaggcgtcctgaaagtgctcagagtgtccctggcacagtttaacaaggcccatgacaatgatggcaatgagcgctacgaccttggcgtaagtgaacgtgtcctgcacacgtgtgccccacttgacataggcacagttcacaaatgtcagcagacatatgcaagcagcagccaggagacggcaggccaggtatgggggatcacagctggggaaggacggctggatgatgtagttggcaaaggtgatggcgatgatggcctgaccggtgggctcaacaactagcagtgagacccacaggcggatgaaggcaatgaagcccccaaaggcctctagaatataagcgtagctggctcccgacttggtgatggtggtccccagctctgcataacaaagggcacccacaacagagaagagcccaccaatggcccacacaatcagtgacatcccataggaggcagtgtgtaccagcacacccttgggtgagacaaagatccctgagccgatcatgttgcccaccaccaggctgaccccattcagcagggagatctccttcttcagctgcatagtttcggaggacctttgaggtggcgagctgacatcttcttccacctgggactggctggtgttagggacaagatggtaggtgggtgtgggcctcccaggctccctggcttccatgacaaacggttcctgcacacctgtgtttgctgtggcctgtaatccccactcaggaggctgaggcaggagaatcgcttgaaccagggagtcggaggttgcagtgagccaagatcacgccactgcctggcaacagagcaagacttggtctgtcaagaaatacgcgaacatcacactttcataagccacctcctcataaatgggtccagtactgagaaggaaatgaagtcccctgcagcaaggcctaattccacttgtctgcctcggccacataaact

SEQ ID NO: 16728 - RNA, 6138 nt, Homo sapiens
  source 1..6138: mol_type = other RNA
taaatttcacctttctgagaagagaaggggctcctgcagtagcctaggaaaatcacatttagaatccactcccgggatgtcattctaggctctgctgactacaacagcctgagtgaggaggaaagaggcagcagcagacagcggatgtggagcaagtaccctctggatgtgcagaaggagttcggctatgacagcccccacgacctggattcagactgatggtcttgtgatgtccatgaggttctgccacatgcccttgagggctctgagtccagagttaactgccctgctgacatcctgttaggtttcctagcttaacatgtggaaggaaaagcatatcaagcatatcgggcggcaccatcccaccacagtgaaaacttatgttaggggagtgagtcttttccacttacagtaggacccctttgcctcaatcaaaagtgaccctacagtttgaaagaaaaaaaaacgttgaaaaaaggaaggtttctttagctttagcttcttggcccaggaatttttcctggcattcaggttctgtgctgaaaccacaagggagggggaggttcccatttcattagcagtaagcttctgctgtgccataccaccaggctgcctgcctctaggaaaaccctgttccttttgatagaatctaaaaggggtaccagtgggtcccttgtagcaatacagactggatagtaatggccattagggcagaaagtagtctgagcagtgggagattttagttaacagctatttctgcttccaaactctgataacggttgtgaaattactgactgacttcctttggcagtggggccaagaaacaatatatatgaatgtgatacatgtgtttagtaaaatctagctttgaacatggaagaaagtaattctttgaaaaccttttaaatctgaatatctaaaacagggagcggtagtgaaatagaaggttcagcattgattataaataccaaggacttaaggcaagggaggaaaaacaaagtaccttctgaacttagctttccactgagtaatgtttactcttcacagcacccaccacaaaaacaaactactatcaacaggatcaattttattaacaacttgtatctcttctaagcagactctgtccgtatgcctttccaaaccatagctgccttaactgactgccttggtgtttattctagcgtaacattgtccagtagaactatctgcagtgatgatatgttctgtgtctgcactgtgtagtagtagacacgggtggctgctgagcacttgaaatgtgattagcgcaactgagaaactgagcttttaattttatttcattttaatgtaattagctacacgtggctagtagctgttgcagcggacaccacaggtctaaggaaacaacacagaacattcagctaggggtgtaccctcatagcctgtgagtgtctcttactcactgtcatgggggaaggtgagttacacagggaggtaccttcttgccgcctcttttaggatttcctaagtatctctccttcatcctacctgccatcattctttgactttatgtccattttctaaacctttgcctacacttgctcttatctacatggagttgttcaacctgccgaagtgattaaattctgtgtacacaggccgtatatattgcagctaattaaaacaacaaacatcctaggcatgcacaaaggtataattcaccgttataacaggcagcaacttgtatgtctaatattagacatcttgctttctgtctgtaggcatagaaacaaaggattgaaagccattctcatacagcaaccgggtgaaaaaaacaaaacactgtgctgttacaatgtgctccctgctatttatactcattaagtttccccaatattaaagggctgacaacttaataaactgtactcactgcaaaagggataataagcacaccaggaaaaggatttaaggagacagacaacaaagagctggcagaaattaattccaccatgaagcttgagtgctgtagggatcctctggcttcgctcccaaagagaggatcctgggagaagtctgtatccagcacagaggggaaaaatgctgtcaccatccaaaaatgaaaggaggatgacatggctcactaagcaagtactagggcacctggcatgtgaggtccttgctttccctagaagccactggtggggggcagcaaattcctgggattagctggttatctggtggagaaagctaaagctggggtcagggatctttaaaaggcaagcacattttgcttaaaggattagctccagaggagccctgggatgggtgccagcttagctcagacagaagtcatgttcttagcgttcaggcaagtcagcctttgcataagacaccctgtcgtcgggcaggaatttgccgttacaaatcccaaacccatgacagtaggaatgtcaccccatgcttcacatatgcattatgctctgaacccagggcaactatgaccatgcttccttcaatctttattgagcaaatatatggccaaggttattcccttatctgtgactgggtggagaagaatggtcaggaagggagactgcctcactgttgaccaattccaaaacctaaggataagcccatggggtatgtcaagctagcaggttcttctcggcccaggatgacagtgtctgggggcatcacaaaacagttgtacaatccaatgcagccgtcctgctcatacagtaagatccattaggccagagcaggcctaacttgggtggagagcccagcctgagcaccagaattagttgcttccacttgtgcagcctgctgaagagccggactcaggttgaagcagctttcctcccagtcttcactgatctccacagggagaaaacagaagtccccacaagtaccaagctcttcctgagactgcagccaccacacctcggggaaggggaggctggcaggagaggagtacactgtcccggtgacccacaccaaggtggctccaagtgtaaacaaagcctggtgccagggacagaagaggatgcagcctgatgtgaggttttcagaaaagtgaaatgacctagcaccaggttgggattgcttgggtctgcacagcagtccctcacactgcccttacagagaggaacaggttatttgatgacttgggcccatgagatgttctccaagccattgacagctgagagaattcaggtgatccacctgaatatcagaagtttcagccctcttagagttcgtaacagaaacccagagatttactgtcagctagaacaaagatgtaaggtctcaagtaaaataaaggattgtccttcaaaacagcaatattaacagacttctgactcaggaatttgttcatctgtccttgctggacctgagccaagtgcttgtaacgtgatctatgatctatctgtatgctaaagtgtaacaggtacgtgagtaaaaaaatctttaaggttcattgttgcaggtaagactcaatagaaattgtgctaaacagcataaaacctgtggtcagagtctgacccaataccacagacatttctgagcccaaagggactcagttttgggtactttgatttttaaatacaatcagcctattgcatcctgtagatgaagagacacgcatgcttcgttagaactggtgttctggactaaatatcaataaataagggaatataactctctccccagggaagaattttgagccagaggaagaaatggtagcatttcaggcctttaaagtcaggtgttgtacctggtcagagaaaaacttcccataaagcagcccctctatagggactcctagttcaaataccaaattcagaagccaccagccctatcaacctagcattccctcttccccactgcactttaccaagtaaatatctgtaagagctgcatctacctatcaggagtaaaactaaatgaccattccccccgttccccaatcttccccccaccctctgaagcccccaccttgaggttggcccagatcctgagtctcctatagcttaccaataagagtgagcactggccctgagccccactatatgattgggtcaaaaggctcctttaattcaggagagttgggcccacagagtcttgttatcaggattttgctggttggcctgccttccaggcctcagaaagccacctctgacctctagtcagttttcctctcatcctttttttcttcggctacatcaagctcagtcaggacacaaaagcaaagctgctgggtgcctctggtgatagcagccaggacattccgaataaacaatggcctccgggactctggcaggtaaacacccatgaagtagaaagggactccagaaagggcaatcccgatgccaatgagggaattaatggtgtcagtgaagaggggcactatcaccagaaacacggagcatatgcagaacacgatggggaaaaacacgctcagcttgagaggccggggccgcttgggctccttccagcggaggtagagctgtccaacaacagacaggcccacgaagaaccagtagctgaagctgaagtagttgataagctggaaaacatcctccacgatgaggtagatgagtgccatggtgcaattgaacagtaaagcagggataggtgtaaaacgctcaatgtggatcatggacagaaggtccggtaggtggccctcccgggagcccacgaagaacaaccttgatgaagcaaagatggatgcattgaggcccccaaagcaggacagggcaacagcaatggggatggtccagctgaacatgccaaacgtctggtcagcaaatgtcacagccacagcatcactgctaaggacatctgaaatgttcagcactgtgtaataggccacattggtcaggatgtagatgagcgtcacaattggcatagaaatcccaatggccaagggcaaatttctttctgggtttttgatttcttctgttacaaaattaagggtgtcccaacctgagtaagagaagagggcagagtagagggcaagagagaggtttcccatgtcccaggaggaaccctcaaaggcgtcctgaaagtgctcagagtgtccctggcacagtttaacaaggcccatgacaatgatggcaatgagcgctacgaccttggcgtaagtgaacgtgtcctgcacacgtgtgccccacttgacataggcacagttcacaaatgtcagcagacatatgcaagcagcagccaggagacggcaggccaggtatgggggatcacagctggggaaggacggctggatgatgtagttggcaaaggtgatggcgatgatggcctgaccggtgggctcaacaactagcagtgagacccacaggcggatgaaggcaatgaagcccccaaaggcctctagaatataagcgtagctggctcccgacttggtgatggtggtccccagctctgcataacaaagggcacccacaacagagaagagcccaccaatggcccacacaatcagtgacatcccataggaggcagtgtgtaccagcacacccttgggtgagacaaagatccctgagccgatcatgttgcccaccaccaggctgaccccattcagcagggagatctccttcttcagctgcatagtttcggaggacctttgaggtggcgagctgacatcttcttccacctgggactggctggtgttagggacaagatggtaggtgggtgtgggcctcccaggctccctggcttccatgacaaacggttcctgcacacctgtgtttgctgtggcctgtaatccccactcaggaggctgaggcaggagaatcgcttgaaccagggagtcggaggttgcagtgagccaagatcacgccactgcctgtcaagaaatacgcgaacatcacactttcataagccacctcctcataaatgggtccagtactgagaaggaaatgaagtcccctgcagcaaggcctaattccacttgtctgcctcggccacataaactccgcagcgcctctcgcgcggccccgatcggccagccccgcgctgtttctgggccgcatcccgctcccgacggcggcagcgaagacccacagggttcggctcccacagaacgcggcccagccccggccccgctcccggcgcgcccgcccatggcccagcccgttacctcccagt

SEQ ID NO: 16729 - RNA, 6016 nt, Homo sapiens
  source 1..6016: mol_type = other RNA
taaatttcacctttctgagaagagaaggggctcctgcagtagcctaggaaaatcacatttagaatccactcccgggatgtcattctaggctctgctgactacaacagcctgagtgaggaggaaagaggcagcagcagacagcggatgtggagcaagtaccctctggatgtgcagaaggagttcggctatgacagcccccacgacctggattcagactgatggtcttgtgatgtccatgaggttctgccacatgcccttgagggctctgagtccagagttaactgccctgctgacatcctgttaggtttcctagcttaacatgtggaaggaaaagcatatcaagcatatcgggcggcaccatcccaccacagtgaaaacttatgttaggggagtgagtcttttccacttacagtaggacccctttgcctcaatcaaaagtgaccctacagtttgaaagaaaaaaaaacgttgaaaaaaggaaggtttctttagctttagcttcttggcccaggaatttttcctggcattcaggttctgtgctgaaaccacaagggagggggaggttcccatttcattagcagtaagcttctgctgtgccataccaccaggctgcctgcctctaggaaaaccctgttccttttgatagaatctaaaaggggtaccagtgggtcccttgtagcaatacagactggatagtaatggccattagggcagaaagtagtctgagcagtgggagattttagttaacagctatttctgcttccaaactctgataacggttgtgaaattactgactgacttcctttggcagtggggccaagaaacaatatatatgaatgtgatacatgtgtttagtaaaatctagctttgaacatggaagaaagtaattctttgaaaaccttttaaatctgaatatctaaaacagggagcggtagtgaaatagaaggttcagcattgattataaataccaaggacttaaggcaagggaggaaaaacaaagtaccttctgaacttagctttccactgagtaatgtttactcttcacagcacccaccacaaaaacaaactactatcaacaggatcaattttattaacaacttgtatctcttctaagcagactctgtccgtatgcctttccaaaccatagctgccttaactgactgccttggtgtttattctagcgtaacattgtccagtagaactatctgcagtgatgatatgttctgtgtctgcactgtgtagtagtagacacgggtggctgctgagcacttgaaatgtgattagcgcaactgagaaactgagcttttaattttatttcattttaatgtaattagctacacgtggctagtagctgttgcagcggacaccacaggtctaaggaaacaacacagaacattcagctaggggtgtaccctcatagcctgtgagtgtctcttactcactgtcatgggggaaggtgagttacacagggaggtaccttcttgccgcctcttttaggatttcctaagtatctctccttcatcctacctgccatcattctttgactttatgtccattttctaaacctttgcctacacttgctcttatctacatggagttgttcaacctgccgaagtgattaaattctgtgtacacaggccgtatatattgcagctaattaaaacaacaaacatcctaggcatgcacaaaggtataattcaccgttataacaggcagcaacttgtatgtctaatattagacatcttgctttctgtctgtaggcatagaaacaaaggattgaaagccattctcatacagcaaccgggtgaaaaaaacaaaacactgtgctgttacaatgtgctccctgctatttatactcattaagtttccccaatattaaagggctgacaacttaataaactgtactcactgcaaaagggataataagcacaccaggaaaaggatttaaggagacagacaacaaagagctggcagaaattaattccaccatgaagcttgagtgctgtagggatcctctggcttcgctcccaaagagaggatcctgggagaagtctgtatccagcacagaggggaaaaatgctgtcaccatccaaaaatgaaaggaggatgacatggctcactaagcaagtactagggcacctggcatgtgaggtccttgctttccctagaagccactggtggggggcagcaaattcctgggattagctggttatctggtggagaaagctaaagctggggtcagggatctttaaaaggcaagcacattttgcttaaaggattagctccagaggagccctgggatgggtgccagcttagctcagacagaagtcatgttcttagcgttcaggcaagtcagcctttgcataagacaccctgtcgtcgggcaggaatttgccgttacaaatcccaaacccatgacagtaggaatgtcaccccatgcttcacatatgcattatgctctgaacccagggcaactatgaccatgcttccttcaatctttattgagcaaatatatggccaaggttattcccttatctgtgactgggtggagaagaatggtcaggaagggagactgcctcactgttgaccaattccaaaacctaaggataagcccatggggtatgtcaagctagcaggttcttctcggcccaggatgacagtgtctgggggcatcacaaaacagttgtacaatccaatgcagccgtcctgctcatacagtaagatccattaggccagagcaggcctaacttgggtggagagcccagcctgagcaccagaattagttgcttccacttgtgcagcctgctgaagagccggactcaggttgaagcagctttcctcccagtcttcactgatctccacagggagaaaacagaagtccccacaagtaccaagctcttcctgagactgcagccaccacacctcggggaaggggaggctggcaggagaggagtacactgtcccggtgacccacaccaaggtggctccaagtgtaaacaaagcctggtgccagggacagaagaggatgcagcctgatgtgaggttttcagaaaagtgaaatgacctagcaccaggttgggattgcttgggtctgcacagcagtccctcacactgcccttacagagaggaacaggttatttgatgacttgggcccatgagatgttctccaagccattgacagctgagagaattcaggtgatccacctgaatatcagaagtttcagccctcttagagttcgtaacagaaacccagagatttactgtcagctagaacaaagatgtaaggtctcaagtaaaataaaggattgtccttcaaaacagcaatattaacagacttctgactcaggaatttgttcatctgtccttgctggacctgagccaagtgcttgtaacgtgatctatgatctatctgtatgctaaagtgtaacaggtacgtgagtaaaaaaatctttaaggttcattgttgcaggtaagactcaatagaaattgtgctaaacagcataaaacctgtggtcagagtctgacccaataccacagacatttctgagcccaaagggactcagttttgggtactttgatttttaaatacaatcagcctattgcatcctgtagatgaagagacacgcatgcttcgttagaactggtgttctggactaaatatcaataaataagggaatataactctctccccagggaagaattttgagccagaggaagaaatggtagcatttcaggcctttaaagtcaggtgttgtacctggtcagagaaaaacttcccataaagcagcccctctatagggactcctagttcaaataccaaattcagaagccaccagccctatcaacctagcattccctcttccccactgcactttaccaagtaaatatctgtaagagctgcatctacctatcaggagtaaaactaaatgaccattccccccgttccccaatcttccccccaccctctgaagcccccaccttgaggttggcccagatcctgagtctcctatagcttaccaataagagtgagcactggccctgagccccactatatgattgggtcaaaaggctcctttaattcaggagagttgggcccacagagtcttgttatcaggattttgctggttggcctgccttccaggcctcagaaagccacctctgacctctagtcagttttcctctcatcctttttttcttcggctacatcaagctcagtcaggacacaaaagcaaagctgctgggtgcctctggtgatagcagccaggacattccgaataaacaatggcctccgggactctggcaggtaaacacccatgaagtagaaagggactccagaaagggcaatcccgatgccaatgagggaattaatggtgtcagtgaagaggggcactatcaccagaaacacggagcatatgcagaacacgatggggaaaaacacgctcagcttgagaggccggggccgcttgggctccttccagcggaggtagagctgtccaacaacagacaggcccacgaagaaccagtagctgaagctgaagtagttgataagctggaaaacatcctccacgatgaggtagatgagtgccatggtgcaattgaacagtaaagcagggataggtgtaaaacgctcaatgtggatcatggacagaaggtccggtaggtggccctcccgggagcccacgaagaacaaccttgatgaagcaaagatggatgcattgaggcccccaaagcaggacagggcaacagcaatggggatggtccagctgaacatgccaaacgtctggtcagcaaatgtcacagccacagcatcactgctaaggacatctgaaatgttcagcactgtgtaataggccacattggtcaggatgtagatgagcgtcacaattggcatagaaatcccaatggccaagggcaaatttctttctgggtttttgatttcttctgttacaaaattaagggtgtcccaacctgagtaagagaagagggcagagtagagggcaagagagaggtttcccatgtcccaggaggaaccctcaaaggcgtcctgaaagtgctcagagtgtccctggcacagtttaacaaggcccatgacaatgatggcaatgagcgctacgaccttggcgtaagtgaacgtgtcctgcacacgtgtgccccacttgacataggcacagttcacaaatgtcagcagacatatgcaagcagcagccaggagacggcaggccaggtatgggggatcacagctggggaaggacggctggatgatgtagttggcaaaggtgatggcgatgatggcctgaccggtgggctcaacaactagcagtgagacccacaggcggatgaaggcaatgaagcccccaaaggcctctagaatataagcgtagctggctcccgacttggtgatggtggtccccagctctgcataacaaagggcacccacaacagagaagagcccaccaatggcccacacaatcagtgacatcccataggaggcagtgtgtaccagcacacccttgggtgagacaaagatccctgagccgatcatgttgcccaccaccaggctgaccccattcagcagggagatctccttcttcagctgcatagtttcggaggacctttgaggtggcgagctgacatcttcttccacctgggactggctggtgttagggacaagatggtaggtgggtgtgggcctcccaggctccctggcttccatgacaaacggttcctgcacacctgtgtttgctgtggcctgtaatccccactcaggaggctgaggcaggagaatcgcttgaaccagggagtcggaggttgcagtgagccaagatcacgccactgcctgtcaagaaatacgcgaacatcacactttcataagccacctcctcataaatgggtccagtactgagaaggaaatgaagtcccctgcagcaaggcctaattccacttgtctgcctcggccacataaactctcccagtggcccggcgccgccaggatgctcggtcgcgccgccgccgccgc

SEQ ID NO: 16730 - RNA, 5961 nt, Homo sapiens
  source 1..5961: mol_type = other RNA
taaatttcacctttctgagaagagaaggggctcctgcagtagcctaggaaaatcacatttagaatccactcccgggatgtcattctaggctctgctgactacaacagcctgagtgaggaggaaagaggcagcagcagacagcggatgtggagcaagtaccctctggatgtgcagaaggagttcggctatgacagcccccacgacctggattcagactgatggtcttgtgatgtccatgaggttctgccacatgcccttgagggctctgagtccagagttaactgccctgctgacatcctgttaggtttcctagcttaacatgtggaaggaaaagcatatcaagcatatcgggcggcaccatcccaccacagtgaaaacttatgttaggggagtgagtcttttccacttacagtaggacccctttgcctcaatcaaaagtgaccctacagtttgaaagaaaaaaaaacgttgaaaaaaggaaggtttctttagctttagcttcttggcccaggaatttttcctggcattcaggttctgtgctgaaaccacaagggagggggaggttcccatttcattagcagtaagcttctgctgtgccataccaccaggctgcctgcctctaggaaaaccctgttccttttgatagaatctaaaaggggtaccagtgggtcccttgtagcaatacagactggatagtaatggccattagggcagaaagtagtctgagcagtgggagattttagttaacagctatttctgcttccaaactctgataacggttgtgaaattactgactgacttcctttggcagtggggccaagaaacaatatatatgaatgtgatacatgtgtttagtaaaatctagctttgaacatggaagaaagtaattctttgaaaaccttttaaatctgaatatctaaaacagggagcggtagtgaaatagaaggttcagcattgattataaataccaaggacttaaggcaagggaggaaaaacaaagtaccttctgaacttagctttccactgagtaatgtttactcttcacagcacccaccacaaaaacaaactactatcaacaggatcaattttattaacaacttgtatctcttctaagcagactctgtccgtatgcctttccaaaccatagctgccttaactgactgccttggtgtttattctagcgtaacattgtccagtagaactatctgcagtgatgatatgttctgtgtctgcactgtgtagtagtagacacgggtggctgctgagcacttgaaatgtgattagcgcaactgagaaactgagcttttaattttatttcattttaatgtaattagctacacgtggctagtagctgttgcagcggacaccacaggtctaaggaaacaacacagaacattcagctaggggtgtaccctcatagcctgtgagtgtctcttactcactgtcatgggggaaggtgagttacacagggaggtaccttcttgccgcctcttttaggatttcctaagtatctctccttcatcctacctgccatcattctttgactttatgtccattttctaaacctttgcctacacttgctcttatctacatggagttgttcaacctgccgaagtgattaaattctgtgtacacaggccgtatatattgcagctaattaaaacaacaaacatcctaggcatgcacaaaggtataattcaccgttataacaggcagcaacttgtatgtctaatattagacatcttgctttctgtctgtaggcatagaaacaaaggattgaaagccattctcatacagcaaccgggtgaaaaaaacaaaacactgtgctgttacaatgtgctccctgctatttatactcattaagtttccccaatattaaagggctgacaacttaataaactgtactcactgcaaaagggataataagcacaccaggaaaaggatttaaggagacagacaacaaagagctggcagaaattaattccaccatgaagcttgagtgctgtagggatcctctggcttcgctcccaaagagaggatcctgggagaagtctgtatccagcacagaggggaaaaatgctgtcaccatccaaaaatgaaaggaggatgacatggctcactaagcaagtactagggcacctggcatgtgaggtccttgctttccctagaagccactggtggggggcagcaaattcctgggattagctggttatctggtggagaaagctaaagctggggtcagggatctttaaaaggcaagcacattttgcttaaaggattagctccagaggagccctgggatgggtgccagcttagctcagacagaagtcatgttcttagcgttcaggcaagtcagcctttgcataagacaccctgtcgtcgggcaggaatttgccgttacaaatcccaaacccatgacagtaggaatgtcaccccatgcttcacatatgcattatgctctgaacccagggcaactatgaccatgcttccttcaatctttattgagcaaatatatggccaaggttattcccttatctgtgactgggtggagaagaatggtcaggaagggagactgcctcactgttgaccaattccaaaacctaaggataagcccatggggtatgtcaagctagcaggttcttctcggcccaggatgacagtgtctgggggcatcacaaaacagttgtacaatccaatgcagccgtcctgctcatacagtaagatccattaggccagagcaggcctaacttgggtggagagcccagcctgagcaccagaattagttgcttccacttgtgcagcctgctgaagagccggactcaggttgaagcagctttcctcccagtcttcactgatctccacagggagaaaacagaagtccccacaagtaccaagctcttcctgagactgcagccaccacacctcggggaaggggaggctggcaggagaggagtacactgtcccggtgacccacaccaaggtggctccaagtgtaaacaaagcctggtgccagggacagaagaggatgcagcctgatgtgaggttttcagaaaagtgaaatgacctagcaccaggttgggattgcttgggtctgcacagcagtccctcacactgcccttacagagaggaacaggttatttgatgacttgggcccatgagatgttctccaagccattgacagctgagagaattcaggtgatccacctgaatatcagaagtttcagccctcttagagttcgtaacagaaacccagagatttactgtcagctagaacaaagatgtaaggtctcaagtaaaataaaggattgtccttcaaaacagcaatattaacagacttctgactcaggaatttgttcatctgtccttgctggacctgagccaagtgcttgtaacgtgatctatgatctatctgtatgctaaagtgtaacaggtacgtgagtaaaaaaatctttaaggttcattgttgcaggtaagactcaatagaaattgtgctaaacagcataaaacctgtggtcagagtctgacccaataccacagacatttctgagcccaaagggactcagttttgggtactttgatttttaaatacaatcagcctattgcatcctgtagatgaagagacacgcatgcttcgttagaactggtgttctggactaaatatcaataaataagggaatataactctctccccagggaagaattttgagccagaggaagaaatggtagcatttcaggcctttaaagtcaggtgttgtacctggtcagagaaaaacttcccataaagcagcccctctatagggactcctagttcaaataccaaattcagaagccaccagccctatcaacctagcattccctcttccccactgcactttaccaagtaaatatctgtaagagctgcatctacctatcaggagtaaaactaaatgaccattccccccgttccccaatcttccccccaccctctgaagcccccaccttgaggttggcccagatcctgagtctcctatagcttaccaataagagtgagcactggccctgagccccactatatgattgggtcaaaaggctcctttaattcaggagagttgggcccacagagtcttgttatcaggattttgctggttggcctgccttccaggcctcagaaagccacctctgacctctagtcagttttcctctcatcctttttttcttcggctacatcaagctcagtcaggacacaaaagcaaagctgctgggtgcctctggtgatagcagccaggacattccgaataaacaatggcctccgggactctggcaggtaaacacccatgaagtagaaagggactccagaaagggcaatcccgatgccaatgagggaattaatggtgtcagtgaagaggggcactatcaccagaaacacggagcatatgcagaacacgatggggaaaaacacgctcagcttgagaggccggggccgcttgggctccttccagcggaggtagagctgtccaacaacagacaggcccacgaagaaccagtagctgaagctgaagtagttgataagctggaaaacatcctccacgatgaggtagatgagtgccatggtgcaattgaacagtaaagcagggataggtgtaaaacgctcaatgtggatcatggacagaaggtccggtaggtggccctcccgggagcccacgaagaacaaccttgatgaagcaaagatggatgcattgaggcccccaaagcaggacagggcaacagcaatggggatggtccagctgaacatgccaaacgtctggtcagcaaatgtcacagccacagcatcactgctaaggacatctgaaatgttcagcactgtgtaataggccacattggtcaggatgtagatgagcgtcacaattggcatagaaatcccaatggccaagggcaaatttctttctgggtttttgatttcttctgttacaaaattaagggtgtcccaacctgagtaagagaagagggcagagtagagggcaagagagaggtttcccatgtcccaggaggaaccctcaaaggcgtcctgaaagtgctcagagtgtccctggcacagtttaacaaggcccatgacaatgatggcaatgagcgctacgaccttggcgtaagtgaacgtgtcctgcacacgtgtgccccacttgacataggcacagttcacaaatgtcagcagacatatgcaagcagcagccaggagacggcaggccaggtatgggggatcacagctggggaaggacggctggatgatgtagttggcaaaggtgatggcgatgatggcctgaccggtgggctcaacaactagcagtgagacccacaggcggatgaaggcaatgaagcccccaaaggcctctagaatataagcgtagctggctcccgacttggtgatggtggtccccagctctgcataacaaagggcacccacaacagagaagagcccaccaatggcccacacaatcagtgacatcccataggaggcagtgtgtaccagcacacccttgggtgagacaaagatccctgagccgatcatgttgcccaccaccaggctgaccccattcagcagggagatctccttcttcagctgcatagtttcggaggacctttgaggtggcgagctgacatcttcttccacctgggactggctggtgttagggacaagatggtaggtgggtgtgggcctcccaggctccctggcttccatgacaaacggttcctgcacacctgtgtttgctgtggcctgtaatccccactcaggaggctgaggcaggagaatcgcttgaaccagggagtcggaggttgcagtgagccaagatcacgccactgtcaagaaatacgcgaacatcacactttcataagccacctcctcataaatgggtccagtactgagaaggaaatgaagtcccctgcagcaaggcctaattccacttgtctgcctcggccacataaact

SEQ ID NO: 16731 - RNA, 6106 nt, Homo sapiens
  source 1..6106: mol_type = other RNA
taaatttcacctttctgagaagagaaggggctcctgcagtagcctaggaaaatcacatttagaatccactcccgggatgtcattctaggctctgctgactacaacagcctgagtgaggaggaaagaggcagcagcagacagcggatgtggagcaagtaccctctggatgtgcagaaggagttcggctatgacagcccccacgacctggattcagactgatggtcttgtgatgtccatgaggttctgccacatgcccttgagggctctgagtccagagttaactgccctgctgacatcctgttaggtttcctagcttaacatgtggaaggaaaagcatatcaagcatatcgggcggcaccatcccaccacagtgaaaacttatgttaggggagtgagtcttttccacttacagtaggacccctttgcctcaatcaaaagtgaccctacagtttgaaagaaaaaaaaacgttgaaaaaaggaaggtttctttagctttagcttcttggcccaggaatttttcctggcattcaggttctgtgctgaaaccacaagggagggggaggttcccatttcattagcagtaagcttctgctgtgccataccaccaggctgcctgcctctaggaaaaccctgttccttttgatagaatctaaaaggggtaccagtgggtcccttgtagcaatacagactggatagtaatggccattagggcagaaagtagtctgagcagtgggagattttagttaacagctatttctgcttccaaactctgataacggttgtgaaattactgactgacttcctttggcagtggggccaagaaacaatatatatgaatgtgatacatgtgtttagtaaaatctagctttgaacatggaagaaagtaattctttgaaaaccttttaaatctgaatatctaaaacagggagcggtagtgaaatagaaggttcagcattgattataaataccaaggacttaaggcaagggaggaaaaacaaagtaccttctgaacttagctttccactgagtaatgtttactcttcacagcacccaccacaaaaacaaactactatcaacaggatcaattttattaacaacttgtatctcttctaagcagactctgtccgtatgcctttccaaaccatagctgccttaactgactgccttggtgtttattctagcgtaacattgtccagtagaactatctgcagtgatgatatgttctgtgtctgcactgtgtagtagtagacacgggtggctgctgagcacttgaaatgtgattagcgcaactgagaaactgagcttttaattttatttcattttaatgtaattagctacacgtggctagtagctgttgcagcggacaccacaggtctaaggaaacaacacagaacattcagctaggggtgtaccctcatagcctgtgagtgtctcttactcactgtcatgggggaaggtgagttacacagggaggtaccttcttgccgcctcttttaggatttcctaagtatctctccttcatcctacctgccatcattctttgactttatgtccattttctaaacctttgcctacacttgctcttatctacatggagttgttcaacctgccgaagtgattaaattctgtgtacacaggccgtatatattgcagctaattaaaacaacaaacatcctaggcatgcacaaaggtataattcaccgttataacaggcagcaacttgtatgtctaatattagacatcttgctttctgtctgtaggcatagaaacaaaggattgaaagccattctcatacagcaaccgggtgaaaaaaacaaaacactgtgctgttacaatgtgctccctgctatttatactcattaagtttccccaatattaaagggctgacaacttaataaactgtactcactgcaaaagggataataagcacaccaggaaaaggatttaaggagacagacaacaaagagctggcagaaattaattccaccatgaagcttgagtgctgtagggatcctctggcttcgctcccaaagagaggatcctgggagaagtctgtatccagcacagaggggaaaaatgctgtcaccatccaaaaatgaaaggaggatgacatggctcactaagcaagtactagggcacctggcatgtgaggtccttgctttccctagaagccactggtggggggcagcaaattcctgggattagctggttatctggtggagaaagctaaagctggggtcagggatctttaaaaggcaagcacattttgcttaaaggattagctccagaggagccctgggatgggtgccagcttagctcagacagaagtcatgttcttagcgttcaggcaagtcagcctttgcataagacaccctgtcgtcgggcaggaatttgccgttacaaatcccaaacccatgacagtaggaatgtcaccccatgcttcacatatgcattatgctctgaacccagggcaactatgaccatgcttccttcaatctttattgagcaaatatatggccaaggttattcccttatctgtgactgggtggagaagaatggtcaggaagggagactgcctcactgttgaccaattccaaaacctaaggataagcccatggggtatgtcaagctagcaggttcttctcggcccaggatgacagtgtctgggggcatcacaaaacagttgtacaatccaatgcagccgtcctgctcatacagtaagatccattaggccagagcaggcctaacttgggtggagagcccagcctgagcaccagaattagttgcttccacttgtgcagcctgctgaagagccggactcaggttgaagcagctttcctcccagtcttcactgatctccacagggagaaaacagaagtccccacaagtaccaagctcttcctgagactgcagccaccacacctcggggaaggggaggctggcaggagaggagtacactgtcccggtgacccacaccaaggtggctccaagtgtaaacaaagcctggtgccagggacagaagaggatgcagcctgatgtgaggttttcagaaaagtgaaatgacctagcaccaggttgggattgcttgggtctgcacagcagtccctcacactgcccttacagagaggaacaggttatttgatgacttgggcccatgagatgttctccaagccattgacagctgagagaattcaggtgatccacctgaatatcagaagtttcagccctcttagagttcgtaacagaaacccagagatttactgtcagctagaacaaagatgtaaggtctcaagtaaaataaaggattgtccttcaaaacagcaatattaacagacttctgactcaggaatttgttcatctgtccttgctggacctgagccaagtgcttgtaacgtgatctatgatctatctgtatgctaaagtgtaacaggtacgtgagtaaaaaaatctttaaggttcattgttgcaggtaagactcaatagaaattgtgctaaacagcataaaacctgtggtcagagtctgacccaataccacagacatttctgagcccaaagggactcagttttgggtactttgatttttaaatacaatcagcctattgcatcctgtagatgaagagacacgcatgcttcgttagaactggtgttctggactaaatatcaataaataagggaatataactctctccccagggaagaattttgagccagaggaagaaatggtagcatttcaggcctttaaagtcaggtgttgtacctggtcagagaaaaacttcccataaagcagcccctctatagggactcctagttcaaataccaaattcagaagccaccagccctatcaacctagcattccctcttccccactgcactttaccaagtaaatatctgtaagagctgcatctacctatcaggagtaaaactaaatgaccattccccccgttccccaatcttccccccaccctctgaagcccccaccttgaggttggcccagatcctgagtctcctatagcttaccaataagagtgagcactggccctgagccccactatatgattgggtcaaaaggctcctttaattcaggagagttgggcccacagagtcttgttatcaggattttgctggttggcctgccttccaggcctcagaaagccacctctgacctctagtcagttttcctctcatcctttttttcttcggctacatcaagctcagtcaggacacaaaagcaaagctgctgggtgcctctggtgatagcagccaggacattccgaataaacaatggcctccgggactctggcaggtaaacacccatgaagtagaaagggactccagaaagggcaatcccgatgccaatgagggaattaatggtgtcagtgaagaggggcactatcaccagaaacacggagcatatgcagaacacgatggggaaaaacacgctcagcttgagaggccggggccgcttgggctccttccagcggaggtagagctgtccaacaacagacaggcccacgaagaaccagtagctgaagctgaagtagttgataagctggaaaacatcctccacgatgaggtagatgagtgccatggtgcaattgaacagtaaagcagggataggtgtaaaacgctcaatgtggatcatggacagaaggtccggtaggtggccctcccgggagcccacgaagaacaaccttgatgaagcaaagatggatgcattgaggcccccaaagcaggacagggcaacagcaatggggatggtccagctgaacatgccaaacgtctggtcagcaaatgtcacagccacagcatcactgctaaggacatctgaaatgttcagcactgtgtaataggccacattggtcaggatgtagatgagcgtcacaattggcatagaaatcccaatggccaagggcaaatttctttctgggtttttgatttcttctgttacaaaattaagggtgtcccaacctgagtaagagaagagggcagagtagagggcaagagagaggtttcccatgtcccaggaggaaccctcaaaggcgtcctgaaagtgctcagagtgtccctggcacagtttaacaaggcccatgacaatgatggcaatgagcgctacgaccttggcgtaagtgaacgtgtcctgcacacgtgtgccccacttgacataggcacagttcacaaatgtcagcagacatatgcaagcagcagccaggagacggcaggccaggtatgggggatcacagctggggaaggacggctggatgatgtagttggcaaaggtgatggcgatgatggcctgaccggtgggctcaacaactagcagtgagacccacaggcggatgaaggcaatgaagcccccaaaggcctctagaatataagcgtagctggctcccgacttggtgatggtggtccccagctctgcataacaaagggcacccacaacagagaagagcccaccaatggcccacacaatcagtgacatcccataggaggcagtgtgtaccagcacacccttgggtgagacaaagatccctgagccgatcatgttgcccaccaccaggctgaccccattcagcagggagatctccttcttcagctgcatagtttcggaggacctttgaggtggcgagctgacatcttcttccacctgggactggctggtgttagggacaagatggtaggtgggtgtgggcctcccaggctccctggcttccatgacaaacggttcctgcacacctgtgtttgctgtggcctgtcaagaaatacgcgaacatcacactttcataagccacctcctcataaatgggtccagtactgagaaggaaatgaagtcccctgcagcaaggcctaattccacttgtctgcctcggccacataaactcaggggcacgcgggttccccagcgccagcagcccaacgctccaggctccagcacgccacaaaaccttgcggcattctctaaagtaaaaggactgattttaaaatgataatcgtcattcttgcgacagccccaggaagcctggctcctgaggtcctgagcccgcgtctttctttgccccaccgcggccgccacacagcacaggttctccgtcctgcagtcggaggcgca

SEQ ID NO: 16732 - RNA, 6041 nt, Homo sapiens
  source 1..6041: mol_type = other RNA
taaatttcacctttctgagaagagaaggggctcctgcagtagcctaggaaaatcacatttagaatccactcccgggatgtcattctaggctctgctgactacaacagcctgagtgaggaggaaagaggcagcagcagacagcggatgtggagcaagtaccctctggatgtgcagaaggagttcggctatgacagcccccacgacctggattcagactgatggtcttgtgatgtccatgaggttctgccacatgcccttgagggctctgagtccagagttaactgccctgctgacatcctgttaggtttcctagcttaacatgtggaaggaaaagcatatcaagcatatcgggcggcaccatcccaccacagtgaaaacttatgttaggggagtgagtcttttccacttacagtaggacccctttgcctcaatcaaaagtgaccctacagtttgaaagaaaaaaaaacgttgaaaaaaggaaggtttctttagctttagcttcttggcccaggaatttttcctggcattcaggttctgtgctgaaaccacaagggagggggaggttcccatttcattagcagtaagcttctgctgtgccataccaccaggctgcctgcctctaggaaaaccctgttccttttgatagaatctaaaaggggtaccagtgggtcccttgtagcaatacagactggatagtaatggccattagggcagaaagtagtctgagcagtgggagattttagttaacagctatttctgcttccaaactctgataacggttgtgaaattactgactgacttcctttggcagtggggccaagaaacaatatatatgaatgtgatacatgtgtttagtaaaatctagctttgaacatggaagaaagtaattctttgaaaaccttttaaatctgaatatctaaaacagggagcggtagtgaaatagaaggttcagcattgattataaataccaaggacttaaggcaagggaggaaaaacaaagtaccttctgaacttagctttccactgagtaatgtttactcttcacagcacccaccacaaaaacaaactactatcaacaggatcaattttattaacaacttgtatctcttctaagcagactctgtccgtatgcctttccaaaccatagctgccttaactgactgccttggtgtttattctagcgtaacattgtccagtagaactatctgcagtgatgatatgttctgtgtctgcactgtgtagtagtagacacgggtggctgctgagcacttgaaatgtgattagcgcaactgagaaactgagcttttaattttatttcattttaatgtaattagctacacgtggctagtagctgttgcagcggacaccacaggtctaaggaaacaacacagaacattcagctaggggtgtaccctcatagcctgtgagtgtctcttactcactgtcatgggggaaggtgagttacacagggaggtaccttcttgccgcctcttttaggatttcctaagtatctctccttcatcctacctgccatcattctttgactttatgtccattttctaaacctttgcctacacttgctcttatctacatggagttgttcaacctgccgaagtgattaaattctgtgtacacaggccgtatatattgcagctaattaaaacaacaaacatcctaggcatgcacaaaggtataattcaccgttataacaggcagcaacttgtatgtctaatattagacatcttgctttctgtctgtaggcatagaaacaaaggattgaaagccattctcatacagcaaccgggtgaaaaaaacaaaacactgtgctgttacaatgtgctccctgctatttatactcattaagtttccccaatattaaagggctgacaacttaataaactgtactcactgcaaaagggataataagcacaccaggaaaaggatttaaggagacagacaacaaagagctggcagaaattaattccaccatgaagcttgagtgctgtagggatcctctggcttcgctcccaaagagaggatcctgggagaagtctgtatccagcacagaggggaaaaatgctgtcaccatccaaaaatgaaaggaggatgacatggctcactaagcaagtactagggcacctggcatgtgaggtccttgctttccctagaagccactggtggggggcagcaaattcctgggattagctggttatctggtggagaaagctaaagctggggtcagggatctttaaaaggcaagcacattttgcttaaaggattagctccagaggagccctgggatgggtgccagcttagctcagacagaagtcatgttcttagcgttcaggcaagtcagcctttgcataagacaccctgtcgtcgggcaggaatttgccgttacaaatcccaaacccatgacagtaggaatgtcaccccatgcttcacatatgcattatgctctgaacccagggcaactatgaccatgcttccttcaatctttattgagcaaatatatggccaaggttattcccttatctgtgactgggtggagaagaatggtcaggaagggagactgcctcactgttgaccaattccaaaacctaaggataagcccatggggtatgtcaagctagcaggttcttctcggcccaggatgacagtgtctgggggcatcacaaaacagttgtacaatccaatgcagccgtcctgctcatacagtaagatccattaggccagagcaggcctaacttgggtggagagcccagcctgagcaccagaattagttgcttccacttgtgcagcctgctgaagagccggactcaggttgaagcagctttcctcccagtcttcactgatctccacagggagaaaacagaagtccccacaagtaccaagctcttcctgagactgcagccaccacacctcggggaaggggaggctggcaggagaggagtacactgtcccggtgacccacaccaaggtggctccaagtgtaaacaaagcctggtgccagggacagaagaggatgcagcctgatgtgaggttttcagaaaagtgaaatgacctagcaccaggttgggattgcttgggtctgcacagcagtccctcacactgcccttacagagaggaacaggttatttgatgacttgggcccatgagatgttctccaagccattgacagctgagagaattcaggtgatccacctgaatatcagaagtttcagccctcttagagttcgtaacagaaacccagagatttactgtcagctagaacaaagatgtaaggtctcaagtaaaataaaggattgtccttcaaaacagcaatattaacagacttctgactcaggaatttgttcatctgtccttgctggacctgagccaagtgcttgtaacgtgatctatgatctatctgtatgctaaagtgtaacaggtacgtgagtaaaaaaatctttaaggttcattgttgcaggtaagactcaatagaaattgtgctaaacagcataaaacctgtggtcagagtctgacccaataccacagacatttctgagcccaaagggactcagttttgggtactttgatttttaaatacaatcagcctattgcatcctgtagatgaagagacacgcatgcttcgttagaactggtgttctggactaaatatcaataaataagggaatataactctctccccagggaagaattttgagccagaggaagaaatggtagcatttcaggcctttaaagtcaggtgttgtacctggtcagagaaaaacttcccataaagcagcccctctatagggactcctagttcaaataccaaattcagaagccaccagccctatcaacctagcattccctcttccccactgcactttaccaagtaaatatctgtaagagctgcatctacctatcaggagtaaaactaaatgaccattccccccgttccccaatcttccccccaccctctgaagcccccaccttgaggttggcccagatcctgagtctcctatagcttaccaataagagtgagcactggccctgagccccactatatgattgggtcaaaaggctcctttaattcaggagagttgggcccacagagtcttgttatcaggattttgctggttggcctgccttccaggcctcagaaagccacctctgacctctagtcagttttcctctcatcctttttttcttcggctacatcaagctcagtcaggacacaaaagcaaagctgctgggtgcctctggtgatagcagccaggacattccgaataaacaatggcctccgggactctggcaggtaaacacccatgaagtagaaagggactccagaaagggcaatcccgatgccaatgagggaattaatggtgtcagtgaagaggggcactatcaccagaaacacggagcatatgcagaacacgatggggaaaaacacgctcagcttgagaggccggggccgcttgggctccttccagcggaggtagagctgtccaacaacagacaggcccacgaagaaccagtagctgaagctgaagtagttgataagctggaaaacatcctccacgatgaggtagatgagtgccatggtgcaattgaacagtaaagcagggataggtgtaaaacgctcaatgtggatcatggacagaaggtccggtaggtggccctcccgggagcccacgaagaacaaccttgatgaagcaaagatggatgcattgaggcccccaaagcaggacagggcaacagcaatggggatggtccagctgaacatgccaaacgtctggtcagcaaatgtcacagccacagcatcactgctaaggacatctgaaatgttcagcactgtgtaataggccacattggtcaggatgtagatgagcgtcacaattggcatagaaatcccaatggccaagggcaaatttctttctgggtttttgatttcttctgttacaaaattaagggtgtcccaacctgagtaagagaagagggcagagtagagggcaagagagaggtttcccatgtcccaggaggaaccctcaaaggcgtcctgaaagtgctcagagtgtccctggcacagtttaacaaggcccatgacaatgatggcaatgagcgctacgaccttggcgtaagtgaacgtgtcctgcacacgtgtgccccacttgacataggcacagttcacaaatgtcagcagacatatgcaagcagcagccaggagacggcaggccaggtatgggggatcacagctggggaaggacggctggatgatgtagttggcaaaggtgatggcgatgatggcctgaccggtgggctcaacaactagcagtgagacccacaggcggatgaaggcaatgaagcccccaaaggcctctagaatataagcgtagctggctcccgacttggtgatggtggtccccagctctgcataacaaagggcacccacaacagagaagagcccaccaatggcccacacaatcagtgacatcccataggaggcagtgtgtaccagcacacccttgggtgagacaaagatccctgagccgatcatgttgcccaccaccaggctgaccccattcagcagggagatctccttcttcagctgcatagtttcggaggacctttgaggtggcgagctgacatcttcttccacctgggactggctggtgttagggacaagatggtaggtgggtgtgggcctcccaggctccctggcttccatgacaaacggttcctgcacacctgtgtttgctgtggcctgtcaagaaatacgcgaacatcacactttcataagccacctcctcataaatgggtccagtactgagaaggaaatgaagtcccctgcagcaaggcctaattccacttgtctgcctcggccacataaactccgcagcgcctctcgcgcggccccgatcggccagccccgcgctgtttctgggccgcatcccgctcccgacggcggcagcgaagacccacagggttcggctcccacagaacgcggcccagccccggccccgctcccggcgcgcccgcccatggcccagcccgtt

SEQ ID NO: 16733 - RNA, 5929 nt, Homo sapiens
  source 1..5929: mol_type = other RNA
taaatttcacctttctgagaagagaaggggctcctgcagtagcctaggaaaatcacatttagaatccactcccgggatgtcattctaggctctgctgactacaacagcctgagtgaggaggaaagaggcagcagcagacagcggatgtggagcaagtaccctctggatgtgcagaaggagttcggctatgacagcccccacgacctggattcagactgatggtcttgtgatgtccatgaggttctgccacatgcccttgagggctctgagtccagagttaactgccctgctgacatcctgttaggtttcctagcttaacatgtggaaggaaaagcatatcaagcatatcgggcggcaccatcccaccacagtgaaaacttatgttaggggagtgagtcttttccacttacagtaggacccctttgcctcaatcaaaagtgaccctacagtttgaaagaaaaaaaaacgttgaaaaaaggaaggtttctttagctttagcttcttggcccaggaatttttcctggcattcaggttctgtgctgaaaccacaagggagggggaggttcccatttcattagcagtaagcttctgctgtgccataccaccaggctgcctgcctctaggaaaaccctgttccttttgatagaatctaaaaggggtaccagtgggtcccttgtagcaatacagactggatagtaatggccattagggcagaaagtagtctgagcagtgggagattttagttaacagctatttctgcttccaaactctgataacggttgtgaaattactgactgacttcctttggcagtggggccaagaaacaatatatatgaatgtgatacatgtgtttagtaaaatctagctttgaacatggaagaaagtaattctttgaaaaccttttaaatctgaatatctaaaacagggagcggtagtgaaatagaaggttcagcattgattataaataccaaggacttaaggcaagggaggaaaaacaaagtaccttctgaacttagctttccactgagtaatgtttactcttcacagcacccaccacaaaaacaaactactatcaacaggatcaattttattaacaacttgtatctcttctaagcagactctgtccgtatgcctttccaaaccatagctgccttaactgactgccttggtgtttattctagcgtaacattgtccagtagaactatctgcagtgatgatatgttctgtgtctgcactgtgtagtagtagacacgggtggctgctgagcacttgaaatgtgattagcgcaactgagaaactgagcttttaattttatttcattttaatgtaattagctacacgtggctagtagctgttgcagcggacaccacaggtctaaggaaacaacacagaacattcagctaggggtgtaccctcatagcctgtgagtgtctcttactcactgtcatgggggaaggtgagttacacagggaggtaccttcttgccgcctcttttaggatttcctaagtatctctccttcatcctacctgccatcattctttgactttatgtccattttctaaacctttgcctacacttgctcttatctacatggagttgttcaacctgccgaagtgattaaattctgtgtacacaggccgtatatattgcagctaattaaaacaacaaacatcctaggcatgcacaaaggtataattcaccgttataacaggcagcaacttgtatgtctaatattagacatcttgctttctgtctgtaggcatagaaacaaaggattgaaagccattctcatacagcaaccgggtgaaaaaaacaaaacactgtgctgttacaatgtgctccctgctatttatactcattaagtttccccaatattaaagggctgacaacttaataaactgtactcactgcaaaagggataataagcacaccaggaaaaggatttaaggagacagacaacaaagagctggcagaaattaattccaccatgaagcttgagtgctgtagggatcctctggcttcgctcccaaagagaggatcctgggagaagtctgtatccagcacagaggggaaaaatgctgtcaccatccaaaaatgaaaggaggatgacatggctcactaagcaagtactagggcacctggcatgtgaggtccttgctttccctagaagccactggtggggggcagcaaattcctgggattagctggttatctggtggagaaagctaaagctggggtcagggatctttaaaaggcaagcacattttgcttaaaggattagctccagaggagccctgggatgggtgccagcttagctcagacagaagtcatgttcttagcgttcaggcaagtcagcctttgcataagacaccctgtcgtcgggcaggaatttgccgttacaaatcccaaacccatgacagtaggaatgtcaccccatgcttcacatatgcattatgctctgaacccagggcaactatgaccatgcttccttcaatctttattgagcaaatatatggccaaggttattcccttatctgtgactgggtggagaagaatggtcaggaagggagactgcctcactgttgaccaattccaaaacctaaggataagcccatggggtatgtcaagctagcaggttcttctcggcccaggatgacagtgtctgggggcatcacaaaacagttgtacaatccaatgcagccgtcctgctcatacagtaagatccattaggccagagcaggcctaacttgggtggagagcccagcctgagcaccagaattagttgcttccacttgtgcagcctgctgaagagccggactcaggttgaagcagctttcctcccagtcttcactgatctccacagggagaaaacagaagtccccacaagtaccaagctcttcctgagactgcagccaccacacctcggggaaggggaggctggcaggagaggagtacactgtcccggtgacccacaccaaggtggctccaagtgtaaacaaagcctggtgccagggacagaagaggatgcagcctgatgtgaggttttcagaaaagtgaaatgacctagcaccaggttgggattgcttgggtctgcacagcagtccctcacactgcccttacagagaggaacaggttatttgatgacttgggcccatgagatgttctccaagccattgacagctgagagaattcaggtgatccacctgaatatcagaagtttcagccctcttagagttcgtaacagaaacccagagatttactgtcagctagaacaaagatgtaaggtctcaagtaaaataaaggattgtccttcaaaacagcaatattaacagacttctgactcaggaatttgttcatctgtccttgctggacctgagccaagtgcttgtaacgtgatctatgatctatctgtatgctaaagtgtaacaggtacgtgagtaaaaaaatctttaaggttcattgttgcaggtaagactcaatagaaattgtgctaaacagcataaaacctgtggtcagagtctgacccaataccacagacatttctgagcccaaagggactcagttttgggtactttgatttttaaatacaatcagcctattgcatcctgtagatgaagagacacgcatgcttcgttagaactggtgttctggactaaatatcaataaataagggaatataactctctccccagggaagaattttgagccagaggaagaaatggtagcatttcaggcctttaaagtcaggtgttgtacctggtcagagaaaaacttcccataaagcagcccctctatagggactcctagttcaaataccaaattcagaagccaccagccctatcaacctagcattccctcttccccactgcactttaccaagtaaatatctgtaagagctgcatctacctatcaggagtaaaactaaatgaccattccccccgttccccaatcttccccccaccctctgaagcccccaccttgaggttggcccagatcctgagtctcctatagcttaccaataagagtgagcactggccctgagccccactatatgattgggtcaaaaggctcctttaattcaggagagttgggcccacagagtcttgttatcaggattttgctggttggcctgccttccaggcctcagaaagccacctctgacctctagtcagttttcctctcatcctttttttcttcggctacatcaagctcagtcaggacacaaaagcaaagctgctgggtgcctctggtgatagcagccaggacattccgaataaacaatggcctccgggactctggcaggtaaacacccatgaagtagaaagggactccagaaagggcaatcccgatgccaatgagggaattaatggtgtcagtgaagaggggcactatcaccagaaacacggagcatatgcagaacacgatggggaaaaacacgctcagcttgagaggccggggccgcttgggctccttccagcggaggtagagctgtccaacaacagacaggcccacgaagaaccagtagctgaagctgaagtagttgataagctggaaaacatcctccacgatgaggtagatgagtgccatggtgcaattgaacagtaaagcagggataggtgtaaaacgctcaatgtggatcatggacagaaggtccggtaggtggccctcccgggagcccacgaagaacaaccttgatgaagcaaagatggatgcattgaggcccccaaagcaggacagggcaacagcaatggggatggtccagctgaacatgccaaacgtctggtcagcaaatgtcacagccacagcatcactgctaaggacatctgaaatgttcagcactgtgtaataggccacattggtcaggatgtagatgagcgtcacaattggcatagaaatcccaatggccaagggcaaatttctttctgggtttttgatttcttctgttacaaaattaagggtgtcccaacctgagtaagagaagagggcagagtagagggcaagagagaggtttcccatgtcccaggaggaaccctcaaaggcgtcctgaaagtgctcagagtgtccctggcacagtttaacaaggcccatgacaatgatggcaatgagcgctacgaccttggcgtaagtgaacgtgtcctgcacacgtgtgccccacttgacataggcacagttcacaaatgtcagcagacatatgcaagcagcagccaggagacggcaggccaggtatgggggatcacagctggggaaggacggctggatgatgtagttggcaaaggtgatggcgatgatggcctgaccggtgggctcaacaactagcagtgagacccacaggcggatgaaggcaatgaagcccccaaaggcctctagaatataagcgtagctggctcccgacttggtgatggtggtccccagctctgcataacaaagggcacccacaacagagaagagcccaccaatggcccacacaatcagtgacatcccataggaggcagtgtgtaccagcacacccttgggtgagacaaagatccctgagccgatcatgttgcccaccaccaggctgaccccattcagcagggagatctccttcttcagctgcatagtttcggaggacctttgaggtggcgagctgacatcttcttccacctgggactggctggtgttagggacaagatggtaggtgggtgtgggcctcccaggctccctggcttccatgacaaacggttcctgcacacctgtgtttgctgtggcctgtcaagaaatacgcgaacatcacactttcataagccacctcctcataaatgggtccagtactgagaaggaaatgaagtcccctgcagcaaggcctaattccacttgtctgcctcggccacataaactctcccagtggcccggcgccgccaggatgctcggtcgcgccgccgccgccgc

SEQ ID NO: 16734 - RNA, 8492 nt, Homo sapiens
  source 1..8492: mol_type = other RNA
taaatttcacctttctgagaagagtaatgtacagcatgcactgcatatgtggtgtccctagggatggggctgtagctgcgagcatggtgatgcctgttttgcatcctgtgcacccactcctcagtgctgggctacttcaaggaactttttgtgccttctagacgactacacataagaactgtggactcctgagaaaacgcatgcactttggttccttaagaatttatctacttttgccaaatgaggcttggctcaaataagaaatacgttgtatagaggccacagccattcttcgtcagctgagacattttactccagattcctcaattctctaaactcttttcactgatcaactagtcatcatttgcaaggattgtcctttagtgctcccaaaaggctctcctgcctctcaggtcccttcattgctgatccacagtgtccattttctgtcaaagactaaaacattttctcattgactgttaaaatacctttcaaagccttcagtcaccaatttatgaagggttaagcatagtccacccaagaatatttcaccctttttaattatcttttttccccattttttaagagtatatttgaagaatggaagggtatgacagaattgatactcaagagatatctcctaggcttctctccccattttcttttggtgacgcttaactcttaacctaatggagagaaatagagggaaataaacacacacacacacacacacacacacacacacacacacacacagagagagagagagagagagagagaggagagagagagagagagaacatgcaagagaaagacaagcaccagactatgtaaggccatctgcagcattaatctagtatacatgtttgggaagtaggttataaataagctatttatattgtggaaatgtgtaaaaaatgttataaatagtaagtgattaatacaattttgattccaactgaaacagaggctacagcataaacaccgaaagggaaaaactataaaaaacaattactatatggttacaggcaggattttggtttatgtttttttagattcagaatgtatgaatatgtataagaccattaatgtctgaaagtaaaaaaaacagttgaagtatcttttccataatgaaaaacattgtaataatagaatacatacaatctttttggggtgggggcaacattctgaacagtaaaaaaattttgtcactttgcaatactgtatgtacatagaattttccaaagtgataactgtttttagtatataatttctaaaactgtattatagtgatgcatgtttacttatataactttaagtgatatcttaaaatgaaataaaagagaatttagttgttatcatacctctgttatgatttctcaaaagaatagtatatttactggtatttgtgttttttttcagtgaaatactgttttgtattactcagccttttttcttccaatttattaaggtttaactgacataaaaatcatatttaaggtgtacaacatgacgttttgatatatgtgtacattatgcaatgattaaatcaagctaattgaaaaataaaatatgaacataaaatatttatttgaaactctaagaaaaaattacaagatctctgtggtaggcagagtaacagcccccgcccaaacaatgttcacaatgtaacccctgaactcgtaagcatcatattttattgtagaagaaaatttgtagatgttattaaatattttgagattgggattatcctagattatctaggtgagcccaacattatcacaagggcccttatacgttggagaaaggtggttagaatgagaaacattgcaaaatactatagtattgactagaggtagaggtaaaggccatgagccaaagaatggagaaagtaactagaatcttctaaagacaatcaagtagattctcctctagagccaacagaaggaacaaagccctgccaatgccttcattttagccaagagaaacctaatttagatttttgacctttagactctaatataataaatttgtgttgttgtaaacaactaaatctgtggcaatttattacagtatcaatagaaaccccaaaacatctgtatgctaaaactgtaaatatactaaaaaaaaatactaattaagtggcgaggactatcatatttatggattgaaggattcaaatctatagacttttagacttccattaatctctagaagtaatacaattccaaccaatgtcccagaaaaatatttgtagacattagcaagatgattctaaaactgatataaaaggcgaataaactagaatatccaaaacaatctgaaagagaatcacaaagctggaaaatttacacttgtaatttccagatttactgtctaattagattacccaatgtactgtggtactgaagaaaggatggacaaatagaaggaccagaaatatccatatatgtcaccaattcattttgactaagctgtaaagtcaatctaatgaagaaatgatagtatttaaacagtaagatgctgggaaatgtgagatatataaaaaatatgaaccttgatcgtatttcaaaccacatacagaaattaacacaatcttaagccaaaacgtcaaactatcaaattgcatgaaaaaaatgagagaaaatatttttgaccattaaattattacatatgatatcaaaatataaaaataaaatttattaaaaataaattgataaaatagactttgaaaaaattaagacgtcttcaaataagaccactgagataataaaaaggcaaattacagaataaaaatatttatcacattattgaattacatataacatatatccagcataaataactacatataatttagcactcctgtgtatactaagtattttactagttactttgtaaaaattatctgtgttttaaaatgtcagttctgttagcatgtgttgaagctgttttgatctgtgttgtagtcctagcacatgaaaaaccctggtttaatgtttacgtattcattctggaccttccttgctatactataatttcgtcacctcgttaatgtgaatatattagtttatcctcataatatataataaattaaaatgtgttcagcttaggagtcaggaacatggaaaggcaagaactctaactgaacaggctgagtatgtatagattcaggaagctcaaaagaggaaaaataactgccaaaaacaacttttacacctgtccgagttattcttatatcagaattctgccaaagaaaactacatttttattgatgtatttctttttcagaccatgaggataattcctatttattacagaacaatgtggaaagcacatacaaggtgtgaaaaacatgaatagcagtaatgaaataattccagtaacatcataatgtggatacagtgtttgataaaatttagatgtggatctttccacacatttatctgtatttatacttaggttttaggatggggtcaacaattttgtgccattttcttataaatgatttcaaataatgcatcatgaatgttttataaaaacattagcctaataattgtgaaacatggttttatgtgctgtttcattctatcatacaatatttttctgattgatttctgacttttttagcattttaaatattttaaatgttttctaagtgttttctactttcagatttactaaaatattccattttaaatagtattttctttttcttagattttgttccataatttttttcattaagaacatacatgtattatcacatttaatccactcaaaaccctcagaaggcagtagttatttttatcatgaacttacagataaagaatgcagcttagagaagttaaataagttgtttaatgctgtgaaccaagtccgtagtctgatcctagggttatactgtaacacgaaaggatacttacacgcaagactaaagaggatcaaacctgatactcaacctatggctgcattccatcctgaaccacagtgccagaaaacagtgattacagttttctatgattcagtgagttcactgggagtttcttctgcttaggctcacctgggctcaaacatgcaactacagacatctactctggggtggtctagaatgccccctcacaaggatgcagttccaactggaatggcaggaacagctagcatggctgggcctctccctccagctggtctttcattctggaattgttctcagcgtggggagctcaagactccaaaagggcaaagacagaaactgtgaaacatcttaggactcagcctaggaaagtgagcaatgtcacatcagaaagatttcactgatcaaaataaccaagccagcatcaccgcataaggaaatgaattcaaaccctgaaaggagagagacaaaaagtctcattgcaaaatggtgttttcacaggaacacctgactcattgggagtcattgttaccaaagcacacacaaaatctacacagtattttcattctagtttacgggatatgtctttgttgttatttgtaaagtgaaacttcacagggttacattgataaaaggtgggggctctctgacaaataccaagaattattaagaatttttgtacttgtgttagcctggatggagcacctttaacatcgctggcacaagtgatatgtttcacttctttaggcacattttttgcttagagttggaaggagcccaggtggtttgctgacccaatagtgctagattgctgagatacttccgagctgactgcttgggaacatggaattgttcatttatgtgtacccattctgggtcaagagactgctgattgcttgggaacactgagagattcctttatgtgtgcccactctgggtcaagacagaccacttgtcctgtgaaccatctggtccaatctctccctgttctctgtgaccttcatgggtagagaggaacaaagcaactaaggctcctgtcattaaccacagttgtcaggtttccttttattgacaaatttggagttggaatggttttgaggagaggagcctgagctgcctgactcaaaccttgcagcaaattcctggctgctctgagacatcttctccctgcagcctgcatcagagggtacatttcagaacagaggcttaaacaatgggaaggaaaagaacaaaaagacaatcaggaatgagtagtaagaataatcggctgccatgctagtcatgggactcaggagaacacaggaggtgaagggtatcacaaatgccttcatcccccaccccagcctacaccactgccagccttgcccctgctctgtccccctcagaaggacaccaagagacagagggtggcaaaaatccaatgcgttattcttttccgaccccctccccactctcaccagatgcctccgaaaatcagctggacggtgggagggatcaagaatgactgccgtcaccatggaaactccttgatggcgagattgctttgagaaccaggaggggatgagataagcaccagaggaacactgggcagtcagggcccagcatccaccaaccctttcttccagataactcctttgttctctgggctggtctccctcttgctcctataggggccctttctgactcttcacctgttttgattcttcagtggtgcccttcccgggtctgggagggaagggcccgaggcccactcagggctgccccaggatggccacttctcactgcagcccagacaccctggtctataagacacactatccttgccactgagaaggaagggacgtcaacacttttgagccaagccctgtgtcccctgcatcctgcaaggaagaagaaaaataaagacctgactatttttcacaggtgcaacgggtgactaaagacagaaagagagtggtgtggttttcacttcatcttgttgagaagccagggcctgaagtccagagatccccattcacatgcaccctcttgggtgggaaggggaggaactcttacctccctctctgccatgttctcctctcgttgcccatttgtgtactatcctccctgtcccctacctgactgcatgtgccttcaatgcaaaggtcttactgctcatcagctttacatctgcatcacagtcacaattcctgcaccttacaggcctggatcaaattcttgtgaatgagcaaaagcatctctaaaggtcaccagtgccctgcttgtctcaatcctagccggacactaggctataatgctcattataaatgtgaaaataaggaaggagaccacctctcccattgtctcctgtttcaaaaaggaagcagaaagttaaaaagaagcagaagtgaggtcaacagccagacagcttggcaccaaaaaccaggcctggtagttaaacatcaactcctaacctaactgcttgtgttatctgtagatgccagacatcgtatgaggaagcgctgtgaaactttctgttctgttctgctagcccccattactgatgcacgtagccctcaatcccatagcccccgcttgcacaatgtatcacgaccctttcacgtggaccccttagagttgtaagcccttaaaagggacaggaatcttcactttggggagctcagaccttgagatgcgagtctactgatgctcccagctgattaaagcctcttccttccttaaactggtgtccgagaggttttgtctgtgaccagtcctgctacaaaagaagctgtgtgcattttttttgcagtgcataaacagactggcctatgatctgtgcctttccttaagtaatatctatcattacaccaaaaatgaaaataaagcctgtggggattatcacgccttccaaatacctgggctgcctctggaggaaactattgctaaatgcccaaagtgaagaaaataaaaaatgtctggagggtagctccccccaaaatactaagaactcctaaataacataaattatggataaatgaaacatctataatcacaggaaatagcataaaatgctattgcaaacccatgattttggtgtatggatagtgtgttcatgtcacttattaaaaccatgaaacctccgggcctggggaaagggaagccgtgcatcccacttgaccagctcatacctccttccttctgcactcagaatcaactgccctttacctgctttcatgccttgatcactactgtttggttctgagatggtgcttttttctgggtggaaattctgcctgaagggagcagggaatttggtgttctaaatccagaaccagcaaaactcaatgagaggggcctcatcccaatgaacccagcacaaacaaacgtgcaacagtcaggcctattttaaaaagacttctcatctctgaacaaatgataccacattttatgaaactcaattacctgcacagtcctttggagaccctgaggctcctgagccttctccaactatcctaggccatcagattaccctactcacactctttaggaaatctgaagttttagattgcttccatcacctgactgaggtcccaagaaggtggctatatgacaaaaaggatccagcctctgcaactgcctattctcctggcaggcctcacctggtgaggccacaaagcatacgagttaaaagaacacagttcctagggacggtggctttggtcggagttctcatgccgacacataatagctacatggcctgaactggttttctaaaacgggaaaggctcagagctcaagcaagatatgagcagaccccatgaaaggtcaacaaatgctggatatggctagacatgtaaggacacaactcagagccatttccttttctcaggttgtaaaacacattttgaggctggagttggggaggtgtgtagctattttgagattggcaataaaactccataaacaccatttacccatgaaattccctgacatgttataaggaaactcacctgagtaggaggaatcaggataaccccccattcaaaactcagggatgtaaaaatatatcacctgctgcccagacacagaggactgctattgctatttagcacaatgtctgcacatcctgtacttgtatctttctctctctctctctcttccctgtgtaaggaaaggcacacaaaaacagttgaaaaaggaaagtcaaaatggcatttctccattctcactaagcctgacctgtctctcctcctttcattccttcacacaattatgtagagaaaaattttaaaacatttttaaaaaatgagcaaagtggcagctactcaccaatttgtgtcctaggcaatccgttgaaccttgattgtgtggtgacgagtgtgctgctgctatcagcctataagctgacatcaaaatgtctacaaaaacctggccaggccccctctcctgccctccctcttccaccttacccagaatgagtgtcccctcacctgagctgagttgtctaagtccatattcaattgataaggagaaatgacactccaagcagcgtcctgttttccaggcaactttttccaaaagctccttttccagaatt

SEQ ID NO: 16735 - RNA, 260 nt, Homo sapiens
  source 1..260: mol_type = other RNA
taaatttcacctttctgagaaggatttttcttgctggattttggaagactatgggtgaccaggactggacacggaattgtagagcttctttatcaggtcagccagggacccgtctaatgccaggttactgggcagtttcgcggagagggcaacaaaggcctctgctattgttgttcccaaaattctatcatccgatctgaccatcacgtcacggtacaacttccaaccgtgcgtccccgaagaggccgggaacggagccc

SEQ ID NO: 16736 - RNA, 218 nt, Homo sapiens
  source 1..218: mol_type = other RNA
taaatttcacctttctgagaaggatttttcttgctggattttggaagactatgggtgaccaggactggacacggaattgtagagcttctttatcaggtcagccagggacccgtctaatgccaggttactgggcagtttcgcggagagggcaacaaaggcctctgctattgttgttcccctgaattctttcttgcgtgagatccaagaaccctctcttg

SEQ ID NO: 16737 - RNA, 256 nt, Homo sapiens
  source 1..256: mol_type = other RNA
taacagtctacagccatggtcgcactctcctgtaaaggcgtcttaaaagagtcaaacccaaagaccttcttcagcgtactccggactcgccgctcagggtcaaaaggaaaggtggtatggtggctgctcatcttagccaagaacacagaaccggccgtggtccgcccaagaattaaaggctgctggctggttccggaactgttcgaagacccctatacacaaccccaactcagagaagccaaagcgctgggaattc

SEQ ID NO: 16738 - RNA, 303 nt, Homo sapiens
  source 1..303: mol_type = other RNA
taacagtctacagccatggtcgcactctcctgtaaaggcgtcttaaaagagtcaaacccaaagaccttcttcagcgtactccggactcgccgctcagggtcaaaaggaaaggtggtatggtggctgctcatcttagccaagaacacagaaccggccgtggtccgcccaagaattaaaggctgctggctggttccggaactgttcgaagacccctatacacaaccccaactcagagaagccaaagcgctgggaattcagctttaggcagaacccacgcaatcttatatccgtcgcgcagtgatg

SEQ ID NO: 16739 - RNA, 304 nt, Homo sapiens
  source 1..304: mol_type = other RNA
taacagtctacagccatggtcgcactctcctgtaaaggcgtcttaaaagagtcaaacccaaagaccttcttcagcgtactccggactcgccgctcagggtcaaaaggaaaggtggtatggtggctgctcatcttagccaagaacacagaaccggccgtggtccgcccaagaattaaaggctgctggctggttccggaactgttcgaagacccctatacacaaccccaactcagagaagccaaagcgctgggaattcagctttaggcagaacccacgcaatcttatatccgtcgcgcagtgatga

SEQ ID NO: 16740 - RNA, 1561 nt, Homo sapiens
  source 1..1561: mol_type = other RNA
taacagtctccagtcacggcccctggagaccggcatgtgggctgtgtgtggggtggagggctgggggtgttggcaagtctcacaggtgaggacccaacgagggaatcagacaaaaagtggccacaaattaggcagctccaggaaggacatgtccttgccatagtaagatgttctgctcacgcgtatccacgagaaagccccgcatttcacggggagcatagaaacaggagtccccaactctgctcaccagctcctccggctgctgccatctgctcctgcagcatggcggcctgggaagcctgcactggtgattttctgccactcaagttttgcagacttcgggaagatggatgcatagcctggggcaatgacagtcacaggcccgccttgtcacaaggtccctggagcgggcaatgccttgagcccaaaggctgggagcacaaagccatcttcagccatcctcgatttccagcaagaccccagggctcacccaacagcccgacactccatactacaaggtgggttaatttttttaaagactctgcagaaatataccaactacagagctcaggaaagcaactgatttataaaacccaatccaagttgtttgcttttatagcattagagacatgtctgaagaacttcaagtttttatctatagaaacataattagtttaataaattactaggtctattttgaataacaaattgagtacttttattagacctaagtggaactttatctgaatctgaattttccaaggggccagtgtagagtgacacaggtgtccgaggccacctttccatcttcagacacccccccgtctctctgcacagggagttggccttccagtaggtgttgctcttctgtcttgacgtctcctggaaagatttttatctctattttcctgtggtggtgttttccacgagctaattctttctatctttaaactcattggctttggaggagctgaattgttagatgacgatctttgtcccaggagagtggcactctgattcttgtggccagcgtatttgggtattgtctcttcatcagctgacagaggtgaaatttttccaaaagcaggttccaatgccagagtgtgcgattcttgccccgcgtgtggggacgctgcagatttcttcctggctttccaccgctgcagctgcagagctctcagcttttctcggagctccatgttctgctccctcaaagcatctatatgactccggagttttccatgaacatcagcccacagagacttctgtctcccaagctcttggtggagtctgatgatctgctgctgtaatggtggcatctccccagtgttgcagtcctccgtgagaacctcggctgccacagctgtcttctccatgacagccccagctcctgggcacgggtcctctgggtgggtgccctctttggggtccctggcctcgagttgacctgccagcatcctggtccccaacagtcactactgccaggatcagatcatctgggccatgtccccacagttgtccccaagccctcctgcctcatatccagagaccagagagcagc

SEQ ID NO: 16741 - RNA, 2113 nt, Homo sapiens
  source 1..2113: mol_type = other RNA
taacagtctccagtcacggcccctggagaccggcatgtgggctgtgtgtggggtggagggctgggggtgttggcaagtctcacaggtgaggacccaacgagggaatcagacaaaaagtggccacaaattaggcagctccaggaaggacatgtccttgccatagtaagatgttctgctcacgcgtatccacgagaaagccccgcatttcacggggagcatagaaacaggagtccccaactctgctcaccagctcctccggctgctgccatctgctcctgcagcatggcggcctgggaagcctgcactggtgattttctgccactcaagttttgcagacttcgggaagatggatgcatagcctggggcaatgacagtcacaggcccgccttgtcacaaggtccctggagcgggcaatgccttgagcccaaaggctgggagcacaaagccatcttcagccatcctcgatttccagcaagaccccagggctcacccaacagcccgacactccatactacaaggtgggttaatttttttaaagactctgcagaaatataccaactacagagctcaggaaagcaactgatttataaaacccaatccaagttgtttgcttttatagcattagagacatgtctgaagaacttcaagtttttatctatagaaacataattagtttaataaattactaggtctattttgaataacaaattgagtacttttattagacctaagtggaactttatctgaatctgaattttccaaggggccagtgtagagtgacacaggtgtccgaggccacctttccatcttcagacacccccccgtctctctgcacagggagttggccttccagtaggtgttgctcttctgtcttgacgtctcctggaaagatttttatctctattttcctgtggtggtgttttccacgagctaattctttctatctttaaactcattggctttggaggagctgaattgttagatgacgatctttgtcccaggagagtggcactctgattcttgtggccagcgtatttgggtattgtctcttcatcagctgacagaggtgaaatttttccaaaagcaggttccaatgccagagtgtgcgattcttgccccgcgtgtggggacgctgcagatttcttcctggctttccaccgctgcagctgcagagctctcagcttttctcggagctccatgttctgctccctcaaagcatctatatgactccggagttttccatgaacatcagcccacagagacttctgtctcccaagctcttggtggagtctgatgatctgctgctgtaatggttgctgaatcttggcgataattttggttttttcattcttccccacgtagtctgaaagcttcttcgttcttctcagctccttggctgcccaccacagctgcgcctctgcctctttaatgacgttgagccctgcctgtgttcccgacaagtcttccttattttcaaactccatgcggatgggatcatacggtggcaaccccatggggtaaacaatcatcaccgcgcctcgaagctggtccaaggcatctttcaccatctccatggtaacacagacaccggcttccacttgtttcttagatattattgctttggcttcttctatagtcttctttaacacttgcttcatcttctcatttggagcttgcccattccttcgtccaatatcatcctttttaaacactgcacctccgctgggtacgcatttttcaccccattcatccttcaatttcaattcttcaatctgatcatcggtcagtccttgcatattaggagggagaaatatgccatgttcggctaattcttccatttctgagcagaggcgctgcaccttgagccgcccattatagacccgggccacctgcaccgtgagctcctccagctcggtactcccaggcgcctgcagcaggaactggctctcgtcgccccgcttcacgtgcagcagaaccatggcggtcccgccgaggtactgaggcgttgagaaggccccggctgcgtggcccgcgggtcctgccggccgagggtcgccggatcgccagcagctgcgacgcactaacagccgctcacagtccggaatcccacgct

SEQ ID NO: 16742 - RNA, 2783 nt, Homo sapiens
  source 1..2783: mol_type = other RNA
taaccctgtcctctccctcccagccaccagtccctcgtccatgtcctcggcaccgggtgcccacctctcatgtgcttcccgttccaagtatccttccaaccggccccatggcccagggtggacggggcttcccggaacccagagggctttcctggcccaggcactggagatccaggaaggggtatggaaggggaggtggggaatgggctgagagaactcgtgccctttcagagctgggtcctcagagctgggggctggggttaccattggccttgggtttggatttgaaggaaaagcgcttgataaggcggcgagaaaagctgccggccttctttcggacactgggcgtggccgttgcgttggagaggtcatcgtgtgattggctcaggccagcttccttctgcctaggcctccggcggaagatgagcttagtgccgctgcgcaggaaactcactgcaggggaagaggggaagctttgtgatccttgaggctgcgggtctccagggcaccagtggaccccgtttccgactcaatatcatccacagatggcctctcagaaatatccgaacgggttgtctcgtctgcttcctggacacttgtgggactagagagggcatctagcggtcctggagacatggctggtgggtctgagggaggtgaagaggggcctccgctggtccctgcatcatcctgcactgaggcttccagggatgccgcatagcccagggatagcgccaactcgtcctgagcaatgggcaccttggaaacaccagagatgatgagagtgctgcgcttggtgggtgtcttcttggccacccgcccactgggctctgtcagctggcgaatcgctgtctctgctacagggtccaagccgttggaaaggtggctgtcccctgggctgctgctatgggaggtattgctggggccactgctctcactcagcacagttgtcgtcttctcggtcacctccaccttggacggggagcgggagggggagtctaatttgccgtctatacggggccgggactggacagtggtgactgtggtgacaatggtgccatcgggcatgatggtccggtcaagctcaatcttcttggtaggtgtgatgctggggcgtggagtggaggaggtgggagtacccaggttccggggagagccctcctcatagtgaagctccactgccatggtggctgctggtcccagggctttccctggccctggggtgagtgggcacaactgtcttcgagacagtggtctggagggggagcccacaggcagtgtggcctggcctaggagttcggtgtctccacagctgctgctcctcagcactttgagggtcagctcccggctctgggggcccagatccagtgccaggtcttctgtccactccacctcggatccagccctcgcgggcttggtccacttctgctgcatggggttgtcgagttcagctacacagcacagttcctcggtgccttccagctcatttcccaagtgagatgcccgaagctgccgtaggaataaccggttaggtctggggatggctggctgagcctggggcatcatgggtggcttctcactgggtaccaggcctcctggggcagagcaagccctgaggttgaccatcatggctggctgggtgctgactatggcatccttgatcagttcctcaattgtggagagctccacttgttcttcacctctctccctggcctgaagcttgggaagcaccgttaggctgagatctgggcgatcagtgaaggcccaggatatgagcagcccctcaccagggatttcctccaggttgacttccaactgtgttggtggcagtgtcagagtgacgtggtaggtctccatggagacggcagcgggggactgctgggtcacagagactgggaaccgcacctcctcagcagagagctggcaacgcagcaccatggtatgctcagattggtctacgcaggtcacatgactgatgctggctctgggtgggagttggggcacctcctcaaaggcgatttggatggagctcccgtttctgcaggcctgctcgttcagcgctcgcacccaagcccgctgccagttctcccggaaagacttgaaggcgaagagtgacgccaggaggccccggactcctggctcctcggcggcgccagcccgagtcgcccgcagccgcagcagcgagcgccacacgcccagctcccgcagggaacccgcgggttccccggctaaggcgggtcccgggccccggtccccgcgggcccgcgccagccacaagccccgggcatattgcagcagccaggcgaacaccgtgagcagcgaggcggcgaagaggatcagcaaggccgcccagcccacgtcccgctgcccccagcccggatccatgctccgcgcgggctccgatcccggtcccggctggggctcacccgctgccccgggggagcatggcccgggcgggccgcggggaggaggtgggctcccccggggctgggcgcgcggggtcgggggctctccgcggctgagtgcccaggactagtgggtgccacagggcgaggagaggaggtcctcgggggtcgcgatgccggggtctctgtctccgtggtccgggtctctcctagcttggtcagcagtcggacccgttagtcgccggccagtgcccgactcctcccaccgcgcgggccccgccggaccctggaggggactggtctgcagagacgctggggctcgcgggccggcaccggctccgggagggctgcgtgcgcagagctgacactgacaacacc

SEQ ID NO: 16743 - RNA, 3329 nt, Homo sapiens
  source 1..3329: mol_type = other RNA
taaccctgtcctctccctcccagccaccagtccctcgtccatgtcctcggcaccgggtgcccacctctcatgtgcttcccgttccaagtatccttccaaccggccccatggcccagggtggacggggcttcccggaacccagagggctttcctggcccaggcactggagatccaggaaggggtatggaaggggaggtggggaatgggctgagagaactcgtgccctttcagagctgggtcctcagagctgggggctggggttaccattggccttgggtttggatttgaaggaaaagcgcttgataaggcggcgagaaaagctgccggccttctttcggacactgggcgtggccgttgcgttggagaggtcatcgtgtgattggctcaggccagcttccttctgcctaggcctccggcggaagatgagcttagtgccgctgcgcaggaaactcactttgtgatccttgaggctgcgggtctccagggcaccagtggaccccgtttccgactcaatatcatccacagatggcctctcagaaatatccgaacgggttgtctcgtctgcttcctggacacttgtgggactagagagggcatctagcggtcctggagacatggctggtgggtctgagggaggtgaagaggggcctccgctggtccctgcatcatcctgcactgaggcttccagggatgccgcatagcccagggatagcgccaactcgtcctgagcaatgggcaccttggaaacaccagagatgatgagagtgctgcgcttggtgggtgtcttcttggccacccgcccactgggctctgtcagctggcgaatcgctgtctctgctacagggtccaagccgttggaaaggtggctgtcccctgggctgctgctatgggaggtattgctggggccactgctctcactcagcacagttgtcgtcttctcggtcacctccacctaatttgccgtctatacggggccgggactggacagtggtgactgtggtgacaatggtgccatcgggcatgatggtccggtcaagctcaatcttcttggtaggtgtgatgctggggcgtggagtggaggaggtgggagtacccaggttccggggagagccctcctcatagtgaagctccactgccatggtggctgctggtcccagggctttccctggccctggggtgagtgggcacaactgtcttcgagacagtggtctggagggggagcccacaggcagtgtggcctggcctaggagttcggtgtctccacagctgctgctcctcagcactttgagggtcagctcccggctctgggggcccagatccagtgccaggtcttctgtccactccacctcggatccagccctcgcgggcttggtccacttctgctgcatggggttgtcgagttcagctacacagcacagttcctcggtgccttccagctcatttcccaagtgagatgcccgaagctgccgtaggaataaccggttaggtctggggatggctggctgagcctggggcatcatgggtggcttctcactgggtaccaggcctcctggggcagagcaagccctgaggttgaccatcatggctggctgggtgctgactatggcatccttgatcagttcctcaattgtggagagctccacttgttcttcacctctctccctggcctgaagcttgggaagcaccgttaggctgagatctgggcgatcagtgaaggcccaggatatgagcagcccctcaccagggatttcctccaggttgacttccaactgtgttggtggcagtgtcagagtgacgtggtaggtctccatggagacggcagcgggggactgctgggtcacagagactgggaaccgcacctcctcagcagagagctggcaacgcagcaccatggtatgctcagattggtctacgcaggtcacatgactgatgctggctctgggtgggagttggggcacctcctcaaaggcgatttggatggagctcccgtttctgcaggcctgctcgttcagcgctcgcacccaagcccgctgccagttctcccggaaagacttgaaggcgaagagtgacgccaggaggccccggactcctggctcctcggcggcgccagcccgagtcgcccgcagccgcagcagcgagcgccacacgcccagctcccgcagggaacccgcgggttccccggctaaggcgggtcccgggccccggtccccgcgggcccgcgccagccacaagccccgggcatattgcagcagccaggcgaacaccgtgagcagcgaggcggcgaagaggatcagcaaggccgcccagcccacgtcccgctgcccccagcccggatccatgctccgcgcgggctccgatcccggtcccggctggggctcacccgctgccccgggggagcatggcccgggcgggccgcggggaggaggtgggctcccccggggctgggcgcgcggggtcgggggctctccgcggctgagtgcccaggactagtgggtgccacagggcgaggagaggaggtcctcgggggtcgcgatgccggggtctctgtctccgtggtccgggtctctcctagcttggtcagcagtcggacccgttagtcgccggccagtgcccgactcctcccaccgcgcgggccccgccggaccctggaggggactggtctgcagagacgctggggctcgcgggccggcaccggctccgggagggctgcgtgcgcagagctgacactgacaacaccgccggcgccccgcccccacccgcccttaaaggagccgcacccgcgccgggcggggccaggacagcctggcgctccctcgctggaggagggcgggagggctagcagcgagcggaggaggttccggggttgaaaataggcgggatctttgatcacctcgccccatcttgcaatcgcggtgctcccacactcagctcaaggcaagagtaacttcacttacctaagatgctgcctttgctttcccctatgcttgttagatttccacaggtcggacgcctgtgaggttaagaaggaggtgacccctgtggaaatcaccgcccccttctcccaacacccccagactcagcgacttctagcttcccatttcctgggggaagctaggcccagggtaaggagacgcagagcgtccctcccagatagaagtgtctggcagaggtccagctgatgtcaacagagagaaagcagaacctgaagctgggagaggttgagagtagaacaccgaatttgaattccccccaccatcatcaccctccttcctcttggagcttggacccagaaacagccccattaacctccttgctcgtgtaggtttgtt

SEQ ID NO: 16744 - RNA, 3154 nt, Homo sapiens
  source 1..3154: mol_type = other RNA
taaccctgtcctctccctcccagccaccagtccctcgtccatgtcctcggcaccgggtgcccacctctcatgtgcttcccgttccaagtatccttccaaccggccccatggcccagggtggacggggcttcccggaacccagagggctttcctggcccaggcactggagatccaggaaggggtatggaaggggaggtggggaatgggctgagagaactcgtgccctttcagagctgggtcctcagagctgggggctggggttaccattggccttgggtttggatttgaaggaaaagcgcttgataaggcggcgagaaaagctgccggccttctttcggacactgggcgtggccgttgcgttggagaggtcatcgtgtgattggctcaggccagcttccttctgcctaggcctccggcggaagatgagcttagtgccgctgcgcaggaaactcactttgtgatccttgaggctgcgggtctccagggcaccagtggaccccgtttccgactcaatatcatccacagatggcctctcagaaatatccgaacgggttgtctcgtctgcttcctggacacttgtgggactagagagggcatctagcggtcctggagacatggctggtgggtctgagggaggtgaagaggggcctccgctggtccctgcatcatcctgcactgaggcttccagggatgccgcatagcccagggatagcgccaactcgtcctgagcaatgggcaccttggaaacaccagagatgatgagagtgctgcgcttggtgggtgtcttcttggccacccgcccactgggctctgtcagctggcgaatcgctgtctctgctacagggtccaagccgttggaaaggtggctgtcccctgggctgctgctatgggaggtattgctggggccactgctctcactcagcacagttgtcgtcttctcggtcacctccacctccactgccatggtggctgctggtcccagggctttccctggccctggggtgagtgggcacaactgtcttcgagacagtggtctggagggggagcccacaggcagtgtggcctggcctaggagttcggtgtctccacagctgctgctcctcagcactttgagggtcagctcccggctctgggggcccagatccagtgccaggtcttctgtccactccacctcggatccagccctcgcgggcttggtccacttctgctgcatggggttgtcgagttcagctacacagcacagttcctcggtgccttccagctcatttcccaagtgagatgcccgaagctgccgtaggaataaccggttaggtctggggatggctggctgagcctggggcatcatgggtggcttctcactgggtaccaggcctcctggggcagagcaagccctgaggttgaccatcatggctggctgggtgctgactatggcatccttgatcagttcctcaattgtggagagctccacttgttcttcacctctctccctggcctgaagcttgggaagcaccgttaggctgagatctgggcgatcagtgaaggcccaggatatgagcagcccctcaccagggatttcctccaggttgacttccaactgtgttggtggcagtgtcagagtgacgtggtaggtctccatggagacggcagcgggggactgctgggtcacagagactgggaaccgcacctcctcagcagagagctggcaacgcagcaccatggtatgctcagattggtctacgcaggtcacatgactgatgctggctctgggtgggagttggggcacctcctcaaaggcgatttggatggagctcccgtttctgcaggcctgctcgttcagcgctcgcacccaagcccgctgccagttctcccggaaagacttgaaggcgaagagtgacgccaggaggccccggactcctggctcctcggcggcgccagcccgagtcgcccgcagccgcagcagcgagcgccacacgcccagctcccgcagggaacccgcgggttccccggctaaggcgggtcccgggccccggtccccgcgggcccgcgccagccacaagccccgggcatattgcagcagccaggcgaacaccgtgagcagcgaggcggcgaagaggatcagcaaggccgcccagcccacgtcccgctgcccccagcccggatccatgctccgcgcgggctccgatcccggtcccggctggggctcacccgctgccccgggggagcatggcccgggcgggccgcggggaggaggtgggctcccccggggctgggcgcgcggggtcgggggctctccgcggctgagtgcccaggactagtgggtgccacagggcgaggagaggaggtcctcgggggtcgcgatgccggggtctctgtctccgtggtccgggtctctcctagcttggtcagcagtcggacccgttagtcgccggccagtgcccgactcctcccaccgcgcgggccccgccggaccctggaggggactggtctgcagagacgctggggctcgcgggccggcaccggctccgggagggctgcgtgcgcagagctgacactgacaacaccgccggcgccccgcccccacccgcccttaaaggagccgcacccgcgccgggcggggccaggacagcctggcgctccctcgctggaggagggcgggagggctagcagcgagcggaggaggttccggggttgaaaataggcgggatctttgatcacctcgccccatcttgcaatcgcggtgctcccacactcagctcaaggcaagagtaacttcacttacctaagatgctgcctttgctttcccctatgcttgttagatttccacaggtcggacgcctgtgaggttaagaaggaggtgacccctgtggaaatcaccgcccccttctcccaacacccccagactcagcgacttctagcttcccatttcctgggggaagctaggcccagggtaaggagacgcagagcgtccctcccagatagaagtgtctggcagaggtccagctgatgtcaacagagagaaagcagaacctgaagctgggagaggttgagagtagaacaccgaatttgaattccccccaccatcatcaccctccttcctcttggagcttggacccagaaacagccccattaacctccttgctcgtgtaggtttgtt

SEQ ID NO: 16745 - RNA, 2763 nt, Homo sapiens
  source 1..2763: mol_type = other RNA
taaccctgtcctctccctcccagccaccagtccctcgtccatgtcctcggcaccgggtgcccacctctcatgtgcttcccgttccaagtatccttccaaccggccccatggcccagggtggacggggcttcccggaacccagagggctttcctggcccaggcactggagatccaggaaggggtatggaaggggaggtggggaatgggctgagagaactcgtgccctttcagagctgggtcctcagagctgggggctggggttaccattggccttgggtttggatttgaaggaaaagcgcttgataaggcggcgagaaaagctgccggccttctttcggacactgggcgtggccgttgcgttggagaggtcatcgtgtgattggctcaggccagcttccttctgcctaggcctccggcggaagatgagcttagtgccgctgcgcaggaaactcactttgtgatccttgaggctgcgggtctccagggcaccagtggaccccgtttccgactcaatatcatccacagatggcctctcagaaatatccgaacgggttgtctcgtctgcttcctggacacttgtgggactagagagggcatctagcggtcctggagacatggctggtgggtctgagggaggtgaagaggggcctccgctggtccctgcatcatcctgcactgaggcttccagggatgccgcatagcccagggatagcgccaactcgtcctgagcaatgggcaccttggaaacaccagagatgatgagagtgctgcgcttggtgggtgtcttcttggccacccgcccactgggctctgtcagctggcgaatcgctgtctctgctacagggtccaagccgttggaaaggtggctgtcccctgggctgctgctatgggaggtattgctggggccactgctctcactcagcacagttgtcgtcttctcggtcacctccaccttggacggggagcgggagggggagtctaatttgccgtctatacggggccgggactggacagtggtgactgtggtgacaatggtgccatcgggcatgatggtccggtcaagctcaatcttcttggtaggtgtgatgctggggcgtggagtggaggaggtgggagtacccaggttccggggagagccctcctcatagtgaagctccactgccatggtggctgctggtcccagggctttccctggccctggggtgagtgggcacaactgtcttcgagacagtggtctggagggggagcccacaggcagtgtggcctggcctaggagttcggtgtctccacagctgctgctcctcagcactttgagggtcagctcccggctctgggggcccagatccagtgccaggtcttctgtccactccacctcggatccagccctcgcgggcttggtccacttctgctgcatggggttgtcgagttcagctacacagcacagttcctcggtgccttccagctcatttcccaagtgagatgcccgaagctgccgtaggaataaccggttaggtctggggatggctggctgagcctggggcatcatgggtggcttctcactgggtaccaggcctcctggggcagagcaagccctgaggttgaccatcatggctggctgggtgctgactatggcatccttgatcagttcctcaattgtggagagctccacttgttcttcacctctctccctggcctgaagcttgggaagcaccgttaggctgagatctgggcgatcagtgaaggcccaggatatgagcagcccctcaccagggatttcctccaggttgacttccaactgtgttggtggcagtgtcagagtgacgtggtaggtctccatggagacggcagcgggggactgctgggtcacagagactgggaaccgcacctcctcagcagagagctggcaacgcagcaccatggtatgctcagattggtctacgcaggtcacatgactgatgctggctctgggtgggagttggggcacctcctcaaaggcgatttggatggagctcccgtttctgcaggcctgctcgttcagcgctcgcacccaagcccgctgccagttctcccggaaagacttgaaggcgaagagtgacgccaggaggccccggactcctggctcctcggcggcgccagcccgagtcgcccgcagccgcagcagcgagcgccacacgcccagctcccgcagggaacccgcgggttccccggctaaggcgggtcccgggccccggtccccgcgggcccgcgccagccacaagccccgggcatattgcagcagccaggcgaacaccgtgagcagcgaggcggcgaagaggatcagcaaggccgcccagcccacgtcccgctgcccccagcccggatccatgctccgcgcgggctccgatcccggtcccggctggggctcacccgctgccccgggggagcatggcccgggcgggccgcggggaggaggtgggctcccccggggctgggcgcgcggggtcgggggctctccgcggctgagtgcccaggactagtgggtgccacagggcgaggagaggaggtcctcgggggtcgcgatgccggggtctctgtctccgtggtccgggtctctcctagcttggtcagcagtcggacccgttagtcgccggccagtgcccgactcctcccaccgcgcgggccccgccggaccctggaggggactggtctgcagagacgctggggctcgcgggccggcaccggctccgggagggctgcgtgcgcagagctgacactgacaacacc

SEQ ID NO: 16746 - RNA, 3254 nt, Homo sapiens
  source 1..3254: mol_type = other RNA
taaccctgtcctctccctcccagccaccagtccctcgtccatgtcctcggcaccgggtgcccacctctcatgtgcttcccgttccaagtatccttccaaccggccccatggcccagggtggacggggcttcccggaacccagagggctttcctggcccaggcactggagatccaggaaggggtatggaaggggaggtggggaatgggctgagagaactcgtgccctttcagagctgggtcctcagagctgggggctggggttaccattggccttgggtttggatttgaaggaaaagcgcttgataaggcggcgagaaaagctgccggccttctttcggacactgggcgtggccgttgcgttggagaggtcatcgtgtgattggctcaggccagcttccttctgcctaggcctccggcggaagatgagcttagtgccgctgcgcaggaaactcactttgtgatccttgaggctgcgggtctccagggcaccagtggaccccgtttccgactcaatatcatccacagatggcctctcagaaatatccgaacgggttgtctcgtctgcttcctggacacttgtgggactagagagggcatctagcggtcctggagacatggctggtgggtctgagggaggtgaagaggggcctccgctggtccctgcatcatcctgcactgaggcttccagggatgccgcatagcccagggatagcgccaactcgtcctgagcaatgggcaccttggaaacaccagagatgatgagagtgctgcgcttggtgggtgtcttcttggccacccgcccactgggctctgtcagctggcgaatcgctgtctctgctacagggtccaagccgttggaaaggtggctgtcccctgggctgctgctatgggaggtattgctggggccactgctctcactcagcacagttgtcgtcttctcggtcacctccaccttggacggggagcgggagggggagtctaatttgccgtctatacggggccgggactggacagtggtgactgtggtgacaatggtgccatcgggcatgatggtccggtcaagctcaatcttcttggtaggtgtgatgctggggcgtggagtggaggaggtgggagtacccaggttccggggagagccctcctcatagtgaagctccactgccatggtggctgctggtcccagggctttccctggccctggggtgagtgggcacaactgtcttcgagacagtggtctggagggggagcccacaggcagtgtggcctggcctaggagttcggtgtctccacagctgctgctcctcagcactttgagggtcagctcccggctctgggggcccagatccagtgccaggtcttctgtccactccacctcggatccagccctcgcgggcttggtccacttctgctgcatggggttgtcgagttcagctacacagcacagttcctcggtgccttccagctcatttcccaagtgagatgcccgaagctgccgtaggaataaccggttaggtctggggatggctggctgagcctggggcatcatgggtggcttctcactgggtaccaggcctcctggggcagagcaagccctgaggttgaccatcatggctggctgggtgctgactatggcatccttgatcagttcctcaattgtggagagctccacttgttcttcacctctctccctggcctgaagcttgggaagcaccgttaggctgagatctgggcgatcagtgaaggcccaggatatgagcagcccctcaccagggatttcctccaggttgacttccaactgtgttggtggcagtgtcagagtgacgtggtaggtctccatggagacggcagcgggggactgctgggtcacagagactgggaaccgcacctcctcagcagagagctggcaacgcagcaccatggtatgctcagattggtctacgcaggtcacatgactgatgctggctctgggtgggagttggggcacctcctcaaaggcgatttggatggagctcgcagccccacctggagagcagtgcggacacagaattgaggaaggggcacagaattggctggcaactcttccttgggtcttgagatggaggaaacaaatccatagggttcatttgcttggcaaaccaggggaagccaactcctttgctctggtagctgtctcattcaaaggctaggccaaggaagatggggagatggatgcttgaaacctcaatctccccaccctctgcaagggaggccaatgtccagttgagtcagctatcctggggagttgcttctgaccgagggacaaggtacagggagagttggatgaagaggtgggttcaaggtgtaaactgacagatgccatctggcttttagccagccagctggacagagtaaatagagcaatttcttgtggacatttctgtttccggcatctggggaactagtaaggtaaagcctccaaactcatagtggctggaaatagagaaccctctgagcaaggagctgatggactgtgagagcaaggagagattgctgggtcaggatgggagggagctccagaaaagagagacttctacctcccaccttatctccatctcatgaccacgcttcctgccccacttcctgggaggccagatgcccatggtgcaatgggaggaagtaggctggactggtttgtgactgaccctcaaggggcagttccaagctcatctactggtaggggcactgtcaatctgctctccacctgaacactccccaacccccagtgaaccacaggccagcatggaggagaaggatgtgtttgactgtagcagtgaaattactgtcgggtaggggggtgattcaggctccttggggatctgcctgaccacaccagggatttggggcatgaaatgttaaatgggtgtggtggcatgagaagcaggcaaattccttctgcaggtgcacctgtctcccatgccccaacacaaccagcacccaggcaaggcggaagtgccctcaggcacagggattagcgttgctatgagaacagcaacttgtgcatgggtttggaaccagagtaccttgcccacagaaatggaagtctggggacccagttggatttctacaacctccagccttagcggcacccttttctctgatccgggaggggaagagaagccatagggttccccagtttatgcccaccctcgtctggcctcctagcacgagcagtcagtccctcccctggaaggaaaggctgaagggaccacccaagc

SEQ ID NO: 16747 - RNA, 3244 nt, Homo sapiens
  source 1..3244: mol_type = other RNA
taaccctgtcctctccctcccagccaccagtccctcgtccatgtcctcggcaccgggtgcccacctctcatgtgcttcccgttccaagtatccttccaaccggccccatggcccagggtggacggggcttcccggaacccagagggctttcctggcccaggcactggagatccaggaaggggtatggaaggggaggtggggaatgggctgagagaactcgtgccctttcagagctgggtcctcagagctgggggctggggttaccattggccttgggtttggatttgaaggaaaagcgcttgataaggcggcgagaaaagctgccggccttctttcggacactgggcgtggccgttgcgttggagaggtcatcgtgtgattggctcaggccagcttccttctgcctaggcctccggcggaagatgagcttagtgccgctgcgcaggaaactcactttgtgatccttgaggctgcgggtctccagggcaccagtggaccccgtttccgactcaatatcatccacagatggcctctcagaaatatccgaacgggttgtctcgtctgcttcctggacacttgtgggactagagagggcatctagcggtcctggagacatggctggtgggtctgagggaggtgaagaggggcctccgctggtccctgcatcatcctgcactgaggcttccagggatgccgcatagcccagggatagcgccaactcgtcctgagcaatgggcaccttggaaacaccagagatgatgagagtgctgcgcttggtgggtgtcttcttggccacccgcccactgggctctgtcagctggcgaatcgctgtctctgctacagggtccaagccgttggaaaggtggctgtcccctgggctgctgctatgggaggtattgctggggccactgctctcactcagcacagttgtcgtcttctcggtcacctccaccttggacggggagcgggagggggagtctaatttgccgtctatacggggccgggactggacagtggtgactgtggtgacaatggtgccatcgggcatgatggtccggtcaagctcaatcttcttggtaggtgtgatgctggggcgtggagtggaggaggtgggagtacccaggttccggggagagccctcctcatagtgaagctccactgccatggtggctgctggtcccagggctttccctggccctggggtgagtgggcacaactgtcttcgagacagtggtctggagggggagcccacaggcagtgtggcctggcctaggagttcggtgtctccacagctgctgctcctcagcactttgagggtcagctcccggctctgggggcccagatccagtgccaggtcttctgtccactccacctcggatccagccctcgcgggcttggtccacttctgctgcatggggttgtcgagttcagctacacagcacagttcctcggtgccttccagctcatttcccaagtgagatgcccgaagctgccgtaggaataaccggttaggtctggggatggctggctgagcctggggcatcatgggtggcttctcactgggtaccaggcctcctggggcagagcaagccctgaggttgaccatcatggctggctgggtgctgactatggcatccttgatcagttcctcaattgtggagagctccacttgttcttcacctctctgtgttggtggcagtgtcagagtgacgtggtaggtctccatggagacggcagcgggggactgctgggtcacagagactgggaaccgcacctcctcagcagagagctggcaacgcagcaccatggtatgctcagattggtctacgcaggtcacatgactgatgctggctctgggtgggagttggggcacctcctcaaaggcgatttggatggagctcccgtttctgcaggcctgctcgttcagcgctcgcacccaagcccgctgccagttctcccggaaagacttgaaggcgaagagtgacgccaggaggccccggactcctggctcctcggcggcgccagcccgagtcgcccgcagccgcagcagcgagcgccacacgcccagctcccgcagggaacccgcgggttccccggctaaggcgggtcccgggccccggtccccgcgggcccgcgccagccacaagccccgggcatattgcagcagccaggcgaacaccgtgagcagcgaggcggcgaagaggatcagcaaggccgcccagcccacgtcccgctgcccccagcccggatccatgctccgcgcgggctccgatcccggtcccggctggggctcacccgctgccccgggggagcatggcccgggcgggccgcggggaggaggtgggctcccccggggctgggcgcgcggggtcgggggctctccgcggctgagtgcccaggactagtgggtgccacagggcgaggagaggaggtcctcgggggtcgcgatgccggggtctctgtctccgtggtccgggtctctcctagcttggtcagcagtcggacccgttagtcgccggccagtgcccgactcctcccaccgcgcgggccccgccggaccctggaggggactggtctgcagagacgctggggctcgcgggccggcaccggctccgggagggctgcgtgcgcagagctgacactgacaacaccgccggcgccccgcccccacccgcccttaaaggagccgcacccgcgccgggcggggccaggacagcctggcgctccctcgctggaggagggcgggagggctagcagcgagcggaggaggttccggggttgaaaataggcgggatctttgatcacctcgccccatcttgcaatcgcggtgctcccacactcagctcaaggcaagagtaacttcacttacctaagatgctgcctttgctttcccctatgcttgttagatttccacaggtcggacgcctgtgaggttaagaaggaggtgacccctgtggaaatcaccgcccccttctcccaacacccccagactcagcgacttctagcttcccatttcctgggggaagctaggcccagggtaaggagacgcagagcgtccctcccagatagaagtgtctggcagaggtccagctgatgtcaacagagagaaagcagaacctgaagctgggagaggttgagagtagaacaccgaatttgaattccccccaccatcatcaccctccttcctcttggagcttggacccagaaacagccccattaacctccttgctcgtgtaggtttgtt

SEQ ID NO: 16748 - RNA, 3326 nt, Homo sapiens
  source 1..3326: mol_type = other RNA
taaccctgtcctctccctcccagccaccagtccctcgtccatgtcctcggcaccgggtgcccacctctcatgtgcttcccgttccaagtatccttccaaccggccccatggcccagggtggacggggcttcccggaacccagagggctttcctggcccaggcactggagatccaggaaggggtatggaaggggaggtggggaatgggctgagagaactcgtgccctttcagagctgggtcctcagagctgggggctggggttaccattggccttgggtttggatttgaaggaaaagcgcttgataaggcggcgagaaaagctgccggccttctttcggacactgggcgtggccgttgcgttggagaggtcatcgtgtgattggctcaggccagcttccttctgcctaggcctccggcggaagatgagcttagtgccgctgcgcaggaaactcactttgtgatccttgaggctgcgggtctccagggcaccagtggaccccgtttccgactcaatatcatccacagatggcctctcagaaatatccgaacgggttgtctcgtctgcttcctggacacttgtgggactagagagggcatctagcggtcctggagacatggctggtgggtctgagggaggtgaagaggggcctccgctggtccctgcatcatcctgcactgaggcttccagggatgccgcatagcccagggatagcgccaactcgtcctgagcaatgggcaccttggaaacaccagagatgatgagagtgctgcgcttggtgggtgtcttcttggccacccgcccactgggctctgtcagctggcgaatcgctgtctctgctacagggtccaagccgttggaaaggtggctgtcccggctgctgctatgggaggtattgctggggccactgctctcactcagcacagttgtcgtcttctcggtcacctccacctaatttgccgtctatacggggccgggactggacagtggtgactgtggtgacaatggtgccatcgggcatgatggtccggtcaagctcaatcttcttggtaggtgtgatgctggggcgtggagtggaggaggtgggagtacccaggttccggggagagccctcctcatagtgaagctccactgccatggtggctgctggtcccagggctttccctggccctggggtgagtgggcacaactgtcttcgagacagtggtctggagggggagcccacaggcagtgtggcctggcctaggagttcggtgtctccacagctgctgctcctcagcactttgagggtcagctcccggctctgggggcccagatccagtgccaggtcttctgtccactccacctcggatccagccctcgcgggcttggtccacttctgctgcatggggttgtcgagttcagctacacagcacagttcctcggtgccttccagctcatttcccaagtgagatgcccgaagctgccgtaggaataaccggttaggtctggggatggctggctgagcctggggcatcatgggtggcttctcactgggtaccaggcctcctggggcagagcaagccctgaggttgaccatcatggctggctgggtgctgactatggcatccttgatcagttcctcaattgtggagagctccacttgttcttcacctctctccctggcctgaagcttgggaagcaccgttaggctgagatctgggcgatcagtgaaggcccaggatatgagcagcccctcaccagggatttcctccaggttgacttccaactgtgttggtggcagtgtcagagtgacgtggtaggtctccatggagacggcagcgggggactgctgggtcacagagactgggaaccgcacctcctcagcagagagctggcaacgcagcaccatggtatgctcagattggtctacgcaggtcacatgactgatgctggctctgggtgggagttggggcacctcctcaaaggcgatttggatggagctcccgtttctgcaggcctgctcgttcagcgctcgcacccaagcccgctgccagttctcccggaaagacttgaaggcgaagagtgacgccaggaggccccggactcctggctcctcggcggcgccagcccgagtcgcccgcagccgcagcagcgagcgccacacgcccagctcccgcagggaacccgcgggttccccggctaaggcgggtcccgggccccggtccccgcgggcccgcgccagccacaagccccgggcatattgcagcagccaggcgaacaccgtgagcagcgaggcggcgaagaggatcagcaaggccgcccagcccacgtcccgctgcccccagcccggatccatgctccgcgcgggctccgatcccggtcccggctggggctcacccgctgccccgggggagcatggcccgggcgggccgcggggaggaggtgggctcccccggggctgggcgcgcggggtcgggggctctccgcggctgagtgcccaggactagtgggtgccacagggcgaggagaggaggtcctcgggggtcgcgatgccggggtctctgtctccgtggtccgggtctctcctagcttggtcagcagtcggacccgttagtcgccggccagtgcccgactcctcccaccgcgcgggccccgccggaccctggaggggactggtctgcagagacgctggggctcgcgggccggcaccggctccgggagggctgcgtgcgcagagctgacactgacaacaccgccggcgccccgcccccacccgcccttaaaggagccgcacccgcgccgggcggggccaggacagcctggcgctccctcgctggaggagggcgggagggctagcagcgagcggaggaggttccggggttgaaaataggcgggatctttgatcacctcgccccatcttgcaatcgcggtgctcccacactcagctcaaggcaagagtaacttcacttacctaagatgctgcctttgctttcccctatgcttgttagatttccacaggtcggacgcctgtgaggttaagaaggaggtgacccctgtggaaatcaccgcccccttctcccaacacccccagactcagcgacttctagcttcccatttcctgggggaagctaggcccagggtaaggagacgcagagcgtccctcccagatagaagtgtctggcagaggtccagctgatgtcaacagagagaaagcagaacctgaagctgggagaggttgagagtagaacaccgaatttgaattccccccaccatcatcaccctccttcctcttggagcttggacccagaaacagccccattaacctccttgctcgtgtaggtttgtt

SEQ ID NO: 16749 - RNA, 3151 nt, Homo sapiens
  source 1..3151: mol_type = other RNA
taaccctgtcctctccctcccagccaccagtccctcgtccatgtcctcggcaccgggtgcccacctctcatgtgcttcccgttccaagtatccttccaaccggccccatggcccagggtggacggggcttcccggaacccagagggctttcctggcccaggcactggagatccaggaaggggtatggaaggggaggtggggaatgggctgagagaactcgtgccctttcagagctgggtcctcagagctgggggctggggttaccattggccttgggtttggatttgaaggaaaagcgcttgataaggcggcgagaaaagctgccggccttctttcggacactgggcgtggccgttgcgttggagaggtcatcgtgtgattggctcaggccagcttccttctgcctaggcctccggcggaagatgagcttagtgccgctgcgcaggaaactcactttgtgatccttgaggctgcgggtctccagggcaccagtggaccccgtttccgactcaatatcatccacagatggcctctcagaaatatccgaacgggttgtctcgtctgcttcctggacacttgtgggactagagagggcatctagcggtcctggagacatggctggtgggtctgagggaggtgaagaggggcctccgctggtccctgcatcatcctgcactgaggcttccagggatgccgcatagcccagggatagcgccaactcgtcctgagcaatgggcaccttggaaacaccagagatgatgagagtgctgcgcttggtgggtgtcttcttggccacccgcccactgggctctgtcagctggcgaatcgctgtctctgctacagggtccaagccgttggaaaggtggctgtcccggctgctgctatgggaggtattgctggggccactgctctcactcagcacagttgtcgtcttctcggtcacctccacctccactgccatggtggctgctggtcccagggctttccctggccctggggtgagtgggcacaactgtcttcgagacagtggtctggagggggagcccacaggcagtgtggcctggcctaggagttcggtgtctccacagctgctgctcctcagcactttgagggtcagctcccggctctgggggcccagatccagtgccaggtcttctgtccactccacctcggatccagccctcgcgggcttggtccacttctgctgcatggggttgtcgagttcagctacacagcacagttcctcggtgccttccagctcatttcccaagtgagatgcccgaagctgccgtaggaataaccggttaggtctggggatggctggctgagcctggggcatcatgggtggcttctcactgggtaccaggcctcctggggcagagcaagccctgaggttgaccatcatggctggctgggtgctgactatggcatccttgatcagttcctcaattgtggagagctccacttgttcttcacctctctccctggcctgaagcttgggaagcaccgttaggctgagatctgggcgatcagtgaaggcccaggatatgagcagcccctcaccagggatttcctccaggttgacttccaactgtgttggtggcagtgtcagagtgacgtggtaggtctccatggagacggcagcgggggactgctgggtcacagagactgggaaccgcacctcctcagcagagagctggcaacgcagcaccatggtatgctcagattggtctacgcaggtcacatgactgatgctggctctgggtgggagttggggcacctcctcaaaggcgatttggatggagctcccgtttctgcaggcctgctcgttcagcgctcgcacccaagcccgctgccagttctcccggaaagacttgaaggcgaagagtgacgccaggaggccccggactcctggctcctcggcggcgccagcccgagtcgcccgcagccgcagcagcgagcgccacacgcccagctcccgcagggaacccgcgggttccccggctaaggcgggtcccgggccccggtccccgcgggcccgcgccagccacaagccccgggcatattgcagcagccaggcgaacaccgtgagcagcgaggcggcgaagaggatcagcaaggccgcccagcccacgtcccgctgcccccagcccggatccatgctccgcgcgggctccgatcccggtcccggctggggctcacccgctgccccgggggagcatggcccgggcgggccgcggggaggaggtgggctcccccggggctgggcgcgcggggtcgggggctctccgcggctgagtgcccaggactagtgggtgccacagggcgaggagaggaggtcctcgggggtcgcgatgccggggtctctgtctccgtggtccgggtctctcctagcttggtcagcagtcggacccgttagtcgccggccagtgcccgactcctcccaccgcgcgggccccgccggaccctggaggggactggtctgcagagacgctggggctcgcgggccggcaccggctccgggagggctgcgtgcgcagagctgacactgacaacaccgccggcgccccgcccccacccgcccttaaaggagccgcacccgcgccgggcggggccaggacagcctggcgctccctcgctggaggagggcgggagggctagcagcgagcggaggaggttccggggttgaaaataggcgggatctttgatcacctcgccccatcttgcaatcgcggtgctcccacactcagctcaaggcaagagtaacttcacttacctaagatgctgcctttgctttcccctatgcttgttagatttccacaggtcggacgcctgtgaggttaagaaggaggtgacccctgtggaaatcaccgcccccttctcccaacacccccagactcagcgacttctagcttcccatttcctgggggaagctaggcccagggtaaggagacgcagagcgtccctcccagatagaagtgtctggcagaggtccagctgatgtcaacagagagaaagcagaacctgaagctgggagaggttgagagtagaacaccgaatttgaattccccccaccatcatcaccctccttcctcttggagcttggacccagaaacagccccattaacctccttgctcgtgtaggtttgtt

SEQ ID NO: 16750 - RNA, 3106 nt, Homo sapiens
  source 1..3106: mol_type = other RNA
taaccctgtcctctccctcccagccaccagtccctcgtccatgtcctcggcaccgggtgcccacctctcatgtgcttcccgttccaagtatccttccaaccggccccatggcccagggtggacggggcttcccggaacccagagggctttcctggcccaggcactggagatccaggaaggggtatggaaggggaggtggggaatgggctgagagaactcgtgccctttcagagctgggtcctcagagctgggggctggggttaccattggccttgggtttggatttgaaggaaaagcgcttgataaggcggcgagaaaagctgccggccttctttcggacactgggcgtggccgttgcgttggagaggtcatcgtgtgattggctcaggccagcttccttctgcctaggcctccggcggaagatgagcttagtgccgctgcgcaggaaactcactttgtgatccttgaggctgcgggtctccagggcaccagtggaccccgtttccgactcaatatcatccacagatggcctctcagaaatatccgaacgggttgtctcgtctgcttcctggacacttgtgggactagagagggcatctagcggtcctggagacatggctggtgggtctgagggaggtgaagaggggcctccgctggtccctgcatcatcctgcactgaggcttccagggatgccgcatagcccagggatagcgccaactcgtcctgagcaatgggcaccttggaaacaccagagatgatgagagtgctgcgcttggtgggtgtcttcttggccacccgcccactgggctctgtcagctggcgaatcgctgtctctgctacagggtccaagccgttggaaaggtggctgtcccggctgctgctatgggaggtattgctggggccactgctctcactcagcacagttgtcgtcttctcggtcacctccaccttggacggggagcgggagggggagtctaatttgccgtctatacggggccgggactggacagtggtgactgtggtgacaatggtgccatcgggcatgatggtccggtcaagctcaatcttcttggtaggtgtgatgctggggcgtggagtggaggaggtgggagtacccaggttccggggagagccctcctcatagtgaagctccactgccatggtggctgctggtcccagggctttccctggccctggggtgagtgggcacaactgtcttcgagacagtggtctggagggggagcccacaggcagtgtggcctggcctaggagttcggtgtctccacagctgctgctcctcagcactttgagggtcagctcccggctctgggggcccagatccagtgccaggtcttctgtccactccacctcggatccagccctcgcgggcttggtccacttctgctgcatggggttgtcgagttcagctacacagcacagttcctcggtgccttccagctcatttcccaagtgagatgcccgaagctgccgtaggaataaccggttaggtctggggatggctggctgagcctggggcatcatgggtggcttctcactgggtaccaggcctcctggggcagagcaagccctgaggttgaccatcatggctggctgggtgctgactatggcatccttgatcagttcctcaattgtggagagctccacttgttcttcacctctctccctggcctgaagcttgggaagcaccgttaggctgagatctgggcgatcagtgaaggcccaggatatgagcagcccctcaccagggatttcctccaggttgacttccaactgtgttggtggcagtgtcagagtgacgtggtaggtctccatggagacggcagcgggggactgctgggtcacagagactgggaaccgcacctcctcagcagagagctggcaacgcagcaccatggtatgctcagattggtctacgcaggtcacatgactgatgctggctctgggtgggagttggggcacctcctcaaaggcgatttggatggagctcccgtttctgcaggcctgctcgttcagcgctcgcacccaagcccgctgccagttctcccggaaagacttgaaggcgaagagtgacgccaggaggccccggactcctggctcctcggcggcgccagcccgagtcgcccgcagccgcagcagcgagcgccacacgcccagctcccgcagggaacccgcgggttccccggctaaggcgggtcccgggccccggtccccgcgggcccgcgccagccacaagccccgggcatattgcagcagccaggcgaacaccgtgagcagcgaggcggcgaagaggatcagcaaggccgcccagcccacgtcccgctgcccccagcccggatccatgctccgcgcgggctccgatcccggtcccggctggggctcacccgctgccccgggggagcatggcccgggcgggccgcggggaggaggtgggctcccccggggctgggcgcgcggggtcgggggctctccgcggctgagtgcccaggactagtgggtgccacagggcgaggagaggaggtcctcgggggtcgcgatgccggggtctctgtctccgtggtccgggtctctcctagcttggtcagcagtcggacccgttagtcgccggccagtgcccgactcctcccaccgcgcgggccccgccggaccctggaggggactggtctgcagagacgctggggctcgcgggccggcaccggctccgggagggctaagatgctgcctttgctttcccctatgcttgttagatttccacaggtcggacgcctgtgaggttaagaaggaggtgacccctgtggaaatcaccgcccccttctcccaacacccccagactcagcgacttctagcttcccatttcctgggggaagctaggcccagggtaaggagacgcagagcgtccctcccagatagaagtgtctggcagaggtccagctgatgtcaacagagagaaagcagaacctgaagctgggagaggttgagagtagaacaccgaatttgaattccccccaccatcatcaccctccttcctcttggagcttggacccagaaacagccccattaacctccttgctcgtgtaggtttgttct

SEQ ID NO: 16751 - RNA, 2760 nt, Homo sapiens
  source 1..2760: mol_type = other RNA
taaccctgtcctctccctcccagccaccagtccctcgtccatgtcctcggcaccgggtgcccacctctcatgtgcttcccgttccaagtatccttccaaccggccccatggcccagggtggacggggcttcccggaacccagagggctttcctggcccaggcactggagatccaggaaggggtatggaaggggaggtggggaatgggctgagagaactcgtgccctttcagagctgggtcctcagagctgggggctggggttaccattggccttgggtttggatttgaaggaaaagcgcttgataaggcggcgagaaaagctgccggccttctttcggacactgggcgtggccgttgcgttggagaggtcatcgtgtgattggctcaggccagcttccttctgcctaggcctccggcggaagatgagcttagtgccgctgcgcaggaaactcactttgtgatccttgaggctgcgggtctccagggcaccagtggaccccgtttccgactcaatatcatccacagatggcctctcagaaatatccgaacgggttgtctcgtctgcttcctggacacttgtgggactagagagggcatctagcggtcctggagacatggctggtgggtctgagggaggtgaagaggggcctccgctggtccctgcatcatcctgcactgaggcttccagggatgccgcatagcccagggatagcgccaactcgtcctgagcaatgggcaccttggaaacaccagagatgatgagagtgctgcgcttggtgggtgtcttcttggccacccgcccactgggctctgtcagctggcgaatcgctgtctctgctacagggtccaagccgttggaaaggtggctgtcccggctgctgctatgggaggtattgctggggccactgctctcactcagcacagttgtcgtcttctcggtcacctccaccttggacggggagcgggagggggagtctaatttgccgtctatacggggccgggactggacagtggtgactgtggtgacaatggtgccatcgggcatgatggtccggtcaagctcaatcttcttggtaggtgtgatgctggggcgtggagtggaggaggtgggagtacccaggttccggggagagccctcctcatagtgaagctccactgccatggtggctgctggtcccagggctttccctggccctggggtgagtgggcacaactgtcttcgagacagtggtctggagggggagcccacaggcagtgtggcctggcctaggagttcggtgtctccacagctgctgctcctcagcactttgagggtcagctcccggctctgggggcccagatccagtgccaggtcttctgtccactccacctcggatccagccctcgcgggcttggtccacttctgctgcatggggttgtcgagttcagctacacagcacagttcctcggtgccttccagctcatttcccaagtgagatgcccgaagctgccgtaggaataaccggttaggtctggggatggctggctgagcctggggcatcatgggtggcttctcactgggtaccaggcctcctggggcagagcaagccctgaggttgaccatcatggctggctgggtgctgactatggcatccttgatcagttcctcaattgtggagagctccacttgttcttcacctctctccctggcctgaagcttgggaagcaccgttaggctgagatctgggcgatcagtgaaggcccaggatatgagcagcccctcaccagggatttcctccaggttgacttccaactgtgttggtggcagtgtcagagtgacgtggtaggtctccatggagacggcagcgggggactgctgggtcacagagactgggaaccgcacctcctcagcagagagctggcaacgcagcaccatggtatgctcagattggtctacgcaggtcacatgactgatgctggctctgggtgggagttggggcacctcctcaaaggcgatttggatggagctcccgtttctgcaggcctgctcgttcagcgctcgcacccaagcccgctgccagttctcccggaaagacttgaaggcgaagagtgacgccaggaggccccggactcctggctcctcggcggcgccagcccgagtcgcccgcagccgcagcagcgagcgccacacgcccagctcccgcagggaacccgcgggttccccggctaaggcgggtcccgggccccggtccccgcgggcccgcgccagccacaagccccgggcatattgcagcagccaggcgaacaccgtgagcagcgaggcggcgaagaggatcagcaaggccgcccagcccacgtcccgctgcccccagcccggatccatgctccgcgcgggctccgatcccggtcccggctggggctcacccgctgccccgggggagcatggcccgggcgggccgcggggaggaggtgggctcccccggggctgggcgcgcggggtcgggggctctccgcggctgagtgcccaggactagtgggtgccacagggcgaggagaggaggtcctcgggggtcgcgatgccggggtctctgtctccgtggtccgggtctctcctagcttggtcagcagtcggacccgttagtcgccggccagtgcccgactcctcccaccgcgcgggccccgccggaccctggaggggactggtctgcagagacgctggggctcgcgggccggcaccggctccgggagggctgcgtgcgcagagctgacactgacaacacc

SEQ ID NO: 16752 - RNA, 2179 nt, Homo sapiens
  source 1..2179: mol_type = other RNA
taaccctgtcctctccctcccagccaccagtccctcgtccatgtcctcggcaccgggtgcccacctctcatgtgcttcccgttccaagtatccttccaaccggccccatggcccagggtggacggggcttcccggaacccagagggctttcctggcccaggcactggagatccaggaaggggtatggaaggggaggtggggaatgggctgagagaactcgtgccctttcagagctgggtcctcagagctgggggctggggttaccattggccttgggtttggatttgaaggaaaagcgcttgataaggcggcgagaaaagctgccggccttctttcggacactgggcgtggccgttgcgttggagaggtcatcgtgtgattggctcaggccagcttccttctgcctaggcctccggcggaagatgagcttagtgccgctgcgcaggaaactcactttgtgatccttgaggctgcgggtctccagggcaccagtggaccccgtttccgactcaatatcatccacagatggcctctcagaaatatccgaacgggttgtctcgtctgcttcctggacacttgtgggactagagagggcatctagcggtcctggagacatggctggtgggtctgagggaggtgaagaggggcctccgctggtccctgcatcatcctgcactgaggcttccagggatgccgcatagcccagggatagcgccaactcgtcctgagcaatgggcaccttggaaacaccagagatgatgagagtgctgcgcttggtgggtgtcttcttggccacccgcccactgggctctgtcagctggcgaatcgctgtctctgctacagggtccaagccgttggaaaggtggctgtcccggctgctgctatgggaggtattgctggggccactgctctcactcagcacagttgtcgtcttctcggtcacctccaccttggacggggagcgggagggggagtctaatttgccgtctatacggggccgggactggacagtggtgactgtggtgacaatggtgccatcgggcatgatggtccggtcaagctcaatcttcttggtaggtgtgatgctggggcgtggagtggaggaggtgggagtacccaggttccggggagagccctcctcatagtgaagctccactgccatggtggctgctggtcccagggctttccctggccctggggtgagtgggcacaactgtcttcgagacagtggtctggagggggagcccacaggcagtgtggcctggcctaggagttcggtgtctccacagctgctgctcctcagcactttgagggtcagctcccggctctgggggcccagatccagtgccaggtcttctgtccactccacctcggatccagccctcgcgggcttggtccacttctgctgcatggggttgtcgagttcagctacacagcacagttcctcggtgccttccagctcatttcccaagtgagatgcccgaagctgccgtaggaataaccggttaggtctggggatggctggctgagcctggggcatcatgggtggcttctcactgggtaccaggcctcctggggcagagcaagccctgaggttgaccatcatggctggctgggtgctgactatggcatccttgatcagttcctcaattgtggagagctccacttgttcttcacctctctccctggcctgaagcttgggaagcaccgttaggctgagatctgggcgatcagtgaaggcccaggatatgagcagcccctcaccagggatttcctccaggttgacttccaactgtgttggtggcagtgtcagagtgacgtggtaggtctccatggagacggcagcgggggactgctgggtcacagagactgggaaccgcacctcctcagcagagagctggcaacgcagcaccatggtatgctcagattggtctacgcaggtcacatgactgatgctggctctgggtgggagttggggcacctcctcaaaggcgatttggatggagctcgcagccccacctggagagcagtgcggacacagaattgaggaaggggcacagaattggctggcaactcttccttgggtcttgagatggaggaaacaaatccatagggttcatttgcttggcaaaccaggggaagccaactcctttgctctggtagctgtctcattcaaagg

SEQ ID NO: 16753 - RNA, 2649 nt, Homo sapiens
  source 1..2649: mol_type = other RNA
taaccctgtcctctccctcccagccaccagtccctcgtccatgtcctcggcaccgggtgcccacctctcatgtgcttcccgttccaagtatccttccaaccggccccatggcccagggtggacggggcttcccggaacccagagggctttcctggcccaggcactggagatccaggaaggggtatggaaggggaggtggggaatgggctgagagaactcgtgccctttcagagctgggtcctcagagctgggggctggggttaccattggccttgggtttggatttgaaggaaaagcgcttgataaggcggcgagaaaagctgccggccttctttcggacactgggcgtggccgttgcgttggagaggtcatcgtgtgattggctcaggccagcttccttctgcctaggcctccggcggaagatgagcttagtgccgctgcgcaggaaactcactttgtgatccttgaggctgcgggtctccagggcaccagtggaccccgtttccgactcaatatcatccacagatggcctctcagaaatatccgaacgggttgtctcgtctgcttcctggacacttgtgggactagagagggcatctagcggtcctggagacatggctggtgggtctgagggaggtgaagaggggcctccgctggtccctgcatcatcctgcactgaggcttccagggatgccgcatagcccagggatagcgccaactcgtcctgagcaatgggcaccttggaaacaccagagatgatgagagtgctgcgcttggtgggtgtcttcttggccacccgcccactgggctctgtcagctggcgaatcgctgtctctgctacagggtccaagccgttggaaaggtggctgtcccggctgctgctatgggaggtattgctggggccactgctctcactcagcacagttgtcgtcttctcggtcacctccaccttggacggggagcgggagggggagtctaatttgccgtctatacggggccgggactggacagtggtgactgtggtgacaatggtgccatcgggcatgatggtccggtcaagctcaatcttcttggtaggtgtgatgctggggcgtggagtggaggaggtgggagtacccaggttccggggagagccctcctcatagtgaagctccactgccatggtggctgctggtcccagggctttccctggccctggggtgagtgggcacaactgtcttcgagacagtggtctggagggggagcccacaggcagtgtggcctggcctaggagttcggtgtctccacagctgctgctcctcagcactttgagggtcagctcccggctctgggggcccagatccagtgccaggtcttctgtccactccacctcggatccagccctcgcgggcttggtccacttctgctgcatggggttgtcgagttcagctacacagcacagttcctcggtgccttccagctcatttcccaagtgagatgcccgaagctgccgtaggaataaccggttaggtctggggatggctggctgagcctggggcatcatgggtggcttctcactgggtaccaggcctcctggggcagagcaagccctgaggttgaccatcatggctggctgggtgctgactatggcatccttgatcagttcctcaattgtggagagctccacttgttcttcacctctctgtgttggtggcagtgtcagagtgacgtggtaggtctccatggagacggcagcgggggactgctgggtcacagagactgggaaccgcacctcctcagcagagagctggcaacgcagcaccatggtatgctcagattggtctacgcaggtcacatgactgatgctggctctgggtgggagttggggcacctcctcaaaggcgatttggatggagctcccgtttctgcaggcctgctcgttcagcgctcgcacccaagcccgctgccagttctcccggaaagacttgaaggcgaagagtgacgccaggaggccccggactcctggctcctcggcggcgccagcccgagtcgcccgcagccgcagcagcgagcgccacacgcccagctcccgcagggaacccgcgggttccccggctaaggcgggtcccgggccccggtccccgcgggcccgcgccagccacaagccccgggcatattgcagcagccaggcgaacaccgtgagcagcgaggcggcgaagaggatcagcaaggccgcccagcccacgtcccgctgcccccagcccggatccatgctccgcgcgggctccgatcccggtcccggctggggctcacccgctgccccgggggagcatggcccgggcgggccgcggggaggaggtgggctcccccggggctgggcgcgcggggtcgggggctctccgcggctgagtgcccaggactagtgggtgccacagggcgaggagaggaggtcctcgggggtcgcgatgccggggtctctgtctccgtggtccgggtctctcctagcttggtcagcagtcggacccgttagtcgccggccagtgcccgactcctcccaccgcgcgggccccgccggaccctggaggggactggtctgcagagacgctggggctcgcgggccggcaccggctccgggagggctgcgtgcgcagagctgacactgacaacacc

SEQ ID NO: 16754 - RNA, 128 nt, Homo sapiens
  source 1..128: mol_type = other RNA
taaccctgtcctctccctcccagccgcagatctgttatggaagggcaggcttctgctctctgccccactccttcaggctggctgattcctcagggtggaaggtggaagggaaggtatggggaagtgga

SEQ ID NO: 16755 - RNA, 48 nt, Homo sapiens
  source 1..48: mol_type = other RNA
taaccctgtcctctccctcccagccgcgacgcgcagggggcgggctct

SEQ ID NO: 16756 - RNA, 148 nt, Homo sapiens
  source 1..148: mol_type = other RNA
taaccctgtcctctccctcccaggccttggcaaccaccagtccgctttctgtctctatggatttacctattctgggcatttcatgtaaatggaatcatacacacgaccttttgtgtctggcttccttcacctagcataatgtatcagg

SEQ ID NO: 16757 - RNA, 4271 nt, Homo sapiens
  source 1..4271: mol_type = other RNA
taacgcataatatggacatgtcaagccataatcaggtttatacggggtaaactaacacctacaaagaacagaaagggtttgctggactatgacataccacagaatggcttaacatttgatacattttagtggtactaattttataactttgggaaacatctgttcatgtaaagcccagcaagggctagtcatcaagtgctagcaatgggagggcagatggtgaggggttaagtgatgtagtcatttgaaaatgtctataaattttccctttaagaggtggagcttaattctccttacccttgaatataggctagacttagtgactccccacttacagaataaggcaaaaatgagcatgtcacttccacagggaggccactgaaaggcactgtggtttccttcttgctttcatactcaggggaaagccagccaccatgctgtgaggacactctatggaagggccgtcaaggagaggaactggggcctctgccctcaaggaaaggaacttaggcctctgccctcaaggagaggaactggggcctctgccctcaagaagaggaactggggcctctgcctaacagccaggtcagtgagcagaaaagtcagccccagtcaaagcatcagatgactgcagccccaaccagtatcttgtttgcaaccttacaccacactctttgccagaaccaccagctaagctgctcccaaattcctgatccagagacctgtgagataaatgtttgctgttttaagacagtaagttttgggatggtttattatatagtaggtaactagtatcggtggtgagcctttggggggtttatgtgaattcatcatgccttgggaaaagcagggtaaagttgaggaaagaaaaggggtataaatgactaaaagagtagatgctgccttgttcaacaagtgcttaaaactagagttaagtgagctctgtgaatatatgagaatgactattaaactctatagccatactactagtactttttatcaattaaagatagtatgaaaggggaaaaaaagctccaaaattgttaatagcatctttattgtttcactggtgcaaaaaaaaaaatcataattgtgatgcatttcctgctaaatttacaatgaaggtgatacataaattatatagatcacaagttttcttttatactatttaaaacccaattatattgataaatatgtccagaggacaacatgggttcttaatggatggctgagtccaaatatgcaaaatatagcttctggttttgaccatggtgctttaaaattctcaaacatgcattaatatattctagttttagggaaaatcttacacatggccttatcttgcaatttaggggaaagcccaagatgaatttcacatacagtattcctttcttctaaattaatctcaaactggactagaaaacaagagacagacgcttttgggttagtactccccaggaatgaagaaaatacacaatcaacaatgaagcaaacaaacaaacaaaaaaaaggagagcttcattagtagccaagataagtgcttgtgggttttgtgtttttttttttttttttttttacagatcacaggaattttaaattgcagatcagtcatgctacttggggtgatcagaaagacttgaacacttaccaagtgaataattttattaaggtcctgaaggtgagtgtccggaggtgctgggtaaaacacatcacaggtaagaaatgggaaacctacctcagcatttctgaaaggcacaatctatggaagggaaacctagcgtaataaaaccctcactggatgtacatggaaaggagtatggtgagctatttcctttttaaaggatgagaccttcataaattggcccctcggattctggtgattcccgccgcaagcgcaaatgctccagtgtgttatgaaaatgtttgttaatctgctctgtttcttcactggattcaagattcgggaggtcttctcgaatcttttggataagctggtttaaaacctgaattgttaccgcatcattttccttttcataaaaatagatatatctgttcagaatttctataaaaagctgcacttgtagagaggggtccatgcactgatttgctatttttagagctttttttaggcactccattaccctcttgcctccgtgaagctcctccccatttttgtccgtgtttctgccagaccagaagagatgtgcacaggtgctcacagctcggccctgatcaggtttctttagaagtttggatgcagcaagggcacactgagtcctcagaggttcgtgattctcttcactgaagcacttcatcctttcaaaagtgccaatgatcaaggtgatggcagctagctgtgctttggaatcgctgatttcatcttcatacagagaaaatgcctgggacatgaattcatatgcgactgtctcatgattttcaaaaccaatttccccagcagctagtgctccttgaagaaaaagtcttaagggcaattctgccagctctgctttgatcaaagcactgatagtctggtgggcaaatgaaaaaatcttctggcatttcttttcccatttgtcatccactttagaattctctttatatcgaaaagccagctggtaagctgcaaataccaaaggtggcagtgtgaagcgaatccgctgatttccaccagctccaaaatgttttcgtgctgtgttcaaaatcaagtactgctggtcagggtcctcagagcgcagcagatgaatgaagcggcccacaaggctctgctcatcagcaaaatcttctggatcagggtcttctacaggttgatctggctgatcttgaatcaacgtggataccaaattcattatggaatccacctggtcttgagagacaatttctgtgttataatccagaacattactaagcacataacaactcatgctctttctggactcgtagtcaaagtactcaaagagtgggtgaaaatgttttaatttcaagactgttaaaatattgttgtaagtgtcaactggtattttcaaaagtctggtgagttcctttgaaactgcactactggtagcaatatgttcaaggttgagcttattgaatatctccactgttgtttctagaactttatcaacatagtccacacgatcagggtaacatttcatggcaagattaatcagagagacttgtaaagatacaacatcctctgaaggcatgtcttgtctagactgtatcactgtagccacctgctgtgaaaatatatcaaaaagtttaatatccgctgggattccaggtccatcttcacggtgagcaaataaagctaatctatcaattaaagcaatgattatgttcttcacatttacattctggtgtaactcagcacaggcccgaagaaaaggattcaaagtctggaggtgaaattcatcagggaaaacctgaataatacactccatgagatattcttgagccaaagcatccctacagtttacaacttgctccaatatgccagtcaaaacaatctgtttgtaacgttccacatttacaccttccaactgactgaggcgcaccaaatttgttcccactaaaattctcagttcttgtctttctcgttctcttttttctctatctcggctatgtccctgatgctgcattcgcacccagagcttgttcatttctgcaaagttgagcagtacaaaatccatggaatcactgatgtcaccagttgtttcttcatctgttggctctccttcatcaggtaagatatttctggtacactgaagaaggtaatttcgaagaaacagacccctcaagggatgttgcacaccacggcacatttctaccaaatctttcaaaatatccttcctggactgaggaaatgacttgacatatacaactccaactgtgatcaaaaggtaaagccttgggataatgtttccagcatactgtacaagttcgtagagatctgccactttccttcctttagcaaactcatctgtcaggtagacctccaagtagtgcagttcatcagaaatggccatataaagttcatagtaactctttggtgataacatagaagtccggagttcaccaagcatattagaagcatgttttagagcatccataagcttgtttttgtccaggcatctcttcatttggaatgactggaccttcacagcctgtatggcttcatccaagagcttttcctgctcatcctgaggggactgctgtgttgtaggcatggcgactccccagagcctgcagcaagcagcacccgccccgcgcgt

SEQ ID NO: 16758 - RNA, 47 nt, Homo sapiens
  source 1..47: mol_type = other RNA
taacgcataatatggacatgttataatttaactgttcattcctctct

SEQ ID NO: 16759 - RNA, 2601 nt, Homo sapiens
  source 1..2601: mol_type = other RNA
taaggggtgtatggcagatgcacctgaatgtgttaggagttccaagtgaggacaagccagagattcattacttacccatgaggaatatctgagcccccattctgtcctgtggatgtacaggggatttagcccctttgttttgggttaaatcaaagttgttagggggagggtgttaagtgaaaatgctatatatactgcatactttctgcaggtggggcagttctcctatctagcccacctccactggactgctctgtatgcaaattcccctcaatcaaacctaagtcttgtttgctggctctggatctcttttggcctctcaaacctggtgccatccctactgaagttaatgggggtctggtggccaggtgcgatggctcacacctataattccagcactttggaaggctgaggcgggtggatcgcctgaggtcaggagttcgtgaccagtctggccctgtctgtactaaaaatacaaaaattagccaggcgtggtggtgtgcgcctgtagtcccagctactcgggaggctgaggcaggagaatggcttgaacccaggaggtggaggttgcagtgagcagagattgcgccactgcactccagcctgagcgacagagcaagactccatctcaaaaaagaaaacaaaacaaaatatgggtctttcttggccgggcgtggtgactcatgctggtaatcccagcattttgggaagctgaggcaggcggatcacctgaggtcaggagttcaagaccagcctggccaatatggtgaaaccccatctgcactaaaaatacaaaaaataagccgggcgtggtggtgcgcacctataatcccagctacttgggaggctgagacacgagaatcgcttgaacctgggaggtggaggttgcagtgagccgagatcgcgtcactgcactccagcctgggcaacagagtaagactgtgtctcaaaaaaacaaacaggccaggcgtggtggctcacgcctgtaatcccagcactttgggaggccaaggcaggcggatcatgaggtcaggaaatccagaccatcctggctaacatggtgaaaccccgtctctactaaaaaatacaaaaaattagctgggcatggtggcgcacgcctgtagtcccagctactctggaggctgaggcaggagaatggcatgaacccgggaggtggagcttgcaatgggccgagatcatgccactgcactccagcctgggcaacagagcaagactccatctcaaaaacaaacccaaacaaacaaaatggccaggtgcagtgcctcacgcctgtaatcccagaactttgggaggctaaggcgggcagatccctaggtcaggagttcgagaccatcctggccaacatggcaaaaccccgtctctactgaaaatacaaaaattaactgggcatggtggcaggtgcctataatcccagctacacaggaggctgatgcaggagaattgcttgaacctgggaggtggaggttgcagtgagctgagatcgtgccattgcactccaccttgggcgacaaaaggaagactccatctaaaagaaaaaaaaaaagccaggtgcggtggctcacgcctgtaatcccagcactttgggaggctgaggcgggtggatcacgaggtcaagagattgagaccatcctggccaacatggagaaaccccatctctactaaaaatagaaaaaatttgctgggtgtggtggtgcacgcctgtagtaccagctacttgggaggctgagacaggagaatcgcttgaacctgggaggcagagcttgcagtgagcagaggtcatgccattgcactccagcctgggcgacagagtgagactcctctcaaaaaaaaataggggcctggcagaacggtcgccctcattccttccagatgccttttgaatgctctgctggatgggtggttggctgagccgtggggcatctgagaacaagtcagtagaccttctccaagagtatgcaataaggactgagcaggaaaaaagttggagactgcctgtcccctcacaaagttgatggtctaacattcttctcagggtcaagaaacttgtccagggagacactgctgtttataatcacaggcctgcttagcctagaacctgggctggcctcttcatcagtggggatgagggctccttgctcccagctgctcagctcccagcagcattgagctcctgggtgtgtgccaagcccgtttgacatctcagagacctgacagactcctgagttattccaccattccacctggcagccaaggtggtcttgactccaccaggcctttgctcttgttgtatgttcagatggctttcctccagatcttcccctgggcgggtcctgctcaggcctcggggctagcttgaatgtcacgccggaaagtgagccctctcttgcccttcatcacagcagaatcacactgatgtgctcgtatgcttctgcttctcgctgtgtctctggtgcttagtaagtgctggccaaaaagaggctcttggcatcagctaattccctggattccctccgtgagctggcatcaggaacactccactgtctcgaccccccgacagcccgagggggcgggtcatctagt

SEQ ID NO: 16760 - RNA, 2680 nt, Homo sapiens
  source 1..2680: mol_type = other RNA
taaggggtgtatggcagatgcacctgaatgtgttaggagttccaagtgaggacaagccagagattcattacttacccatgaggaatatctgagcccccattctgtcctgtggatgtacaggggatttagcccctttgttttgggttaaatcaaagttgttagggggagggtgttaagtgaaaatgctatatatactgcatactttctgcaggtggggcagttctcctatctagcccacctccactggactgctctgtatgcaaattcccctcaatcaaacctaagtcttgtttgctggctctggatctcttttggcctctcaaacctggtgccatccctactgaagttaatgggggtctggtggccaggtgcgatggctcacacctataattccagcactttggaaggctgaggcgggtggatcgcctgaggtcaggagttcgtgaccagtctggccctgtctgtactaaaaatacaaaaattagccaggcgtggtggtgtgcgcctgtagtcccagctactcgggaggctgaggcaggagaatggcttgaacccaggaggtggaggttgcagtgagcagagattgcgccactgcactccagcctgagcgacagagcaagactccatctcaaaaaagaaaacaaaacaaaatatgggtctttcttggccgggcgtggtgactcatgctggtaatcccagcattttgggaagctgaggcaggcggatcacctgaggtcaggagttcaagaccagcctggccaatatggtgaaaccccatctgcactaaaaatacaaaaaataagccgggcgtggtggtgcgcacctataatcccagctacttgggaggctgagacacgagaatcgcttgaacctgggaggtggaggttgcagtgagccgagatcgcgtcactgcactccagcctgggcaacagagtaagactgtgtctcaaaaaaacaaacaggccaggcgtggtggctcacgcctgtaatcccagcactttgggaggccaaggcaggcggatcatgaggtcaggaaatccagaccatcctggctaacatggtgaaaccccgtctctactaaaaaatacaaaaaattagctgggcatggtggcgcacgcctgtagtcccagctactctggaggctgaggcaggagaatggcatgaacccgggaggtggagcttgcaatgggccgagatcatgccactgcactccagcctgggcaacagagcaagactccatctcaaaaacaaacccaaacaaacaaaatggccaggtgcagtgcctcacgcctgtaatcccagaactttgggaggctaaggcgggcagatccctaggtcaggagttcgagaccatcctggccaacatggcaaaaccccgtctctactgaaaatacaaaaattaactgggcatggtggcaggtgcctataatcccagctacacaggaggctgatgcaggagaattgcttgaacctgggaggtggaggttgcagtgagctgagatcgtgccattgcactccaccttgggcgacaaaaggaagactccatctaaaagaaaaaaaaaaagccaggtgcggtggctcacgcctgtaatcccagcactttgggaggctgaggcgggtggatcacgaggtcaagagattgagaccatcctggccaacatggagaaaccccatctctactaaaaatagaaaaaatttgctgggtgtggtggtgcacgcctgtagtaccagctacttgggaggctgagacaggagaatcgcttgaacctgggaggcagagcttgcagtgagcagaggtcatgccattgcactccagcctgggcgacagagtgagactcctctcaaaaaaaaataggggcctggcagaacggtcgccctcattccttccagatgccttttgaatgctctgctggatgggtggttggctgagccgtggggcatctgagaacaagtcagtagaccttctccaagagtatgcaataaggactgagcaggaaaaaagttggagactgcctgtcccctcacaaagttgatggtctaacattcttctcagggtcaagaaacttgtccagggagacactgctgtttataatcacaggcctgcttagcctagaacctgggctggcctcttcatcagtggggatgagggctccttgctcccagctgctcagctcccagcagcattgagctcctgggtgtgtgccaagcccgtttgacatctcagagacctgacagactcctgagttattccaccattccacctggcagccaaggtggtcttgactccaccaggcctttgctcttgttgtatgttcagatggctttcctccagatcttcccctgggcgggtcctgctcaggcctcggggctagcttgaatgtcacgccggaaagtgagccctctcttgcccttcatcacagcagaatcacactgatgtgctcgtatgcttctgcttctcgctgtgtctctggtgcttagtaagtgctggccaaaaagaggctcttggcatcagctgaaagaataatttaaaggtcttcaggaccaggcgagaggcactaatcggtccccttcatgggtagaccgttcattacctaattccctggattccctccgtgagctggcatcaggaacactccactgtctcgaccccccgacagcccgagggggcgggtcatctagt

SEQ ID NO: 16761 - RNA, 2551 nt, Homo sapiens
  source 1..2551: mol_type = other RNA
taaggggtgtatggcagatgcatctgacagcaataacttaagaagtgagggttgccacgtggaggctgctgaggggagggtgctgagtgaaagtgctatgtaaactgcatgctttttataagtggttgcagttctgtccagcccgcggccactggaccaccctgtaaggttccccaaataaaccctatgtttccttcactagctccaggtctcttctttggcctcttgaacctggtgccatccctactgaagttaacagaggtctggcccaacctaagggcatcattttttaaagtcccatggaaaaaactcccagcagagttcagcatctgggaacggttggcaggccccacaggaaccacagcttctgcctttatgatgctgagaaacacttcactgttgacttcccccatctaagggggccagagctaaattttgggcagctgtgtttatcctgggggtccacatatttgcatcattctttcttctcatcgtgatgttctaccttgttggtactgttctcttccttctttgtgtgagttcctgttgtgagcttccccttgttcactgaggtaatgtagccaaacaaggttaaaaagcccccagtaagccgggtgcggtggctcatgcccgtaatctcagcactttgggaggccgaggcgggcagatcacctgaggtcgagagtttaagaccagcctgaccaacatggagaaaccccgtctctactaaaaatacaaaattagctgggtgtggtggtacatacctgtaatcccagctactcatgaggctgaggcaggagaatctcttgaacccgggaggcggaggttgctgtgagctgagatcgcaccactgcactccagcctgggcaacaagagtgaaactctgtctcaaaaaaaaaaaaaaaaagtccctaataaagccatatcgtggggtaatgtctttatacaataaattacctactgtagagtgtgattttattttccactaaaacttgtgcaaaaatcagaatagtagggtttttaccccttgacttctactttgcccagataacaaaaatataatcagaataactattttttttagacaatctaatttacaaaatttttccctcccaataaccaaccatacacatcaaagatacctcacgtttcagttcaaaccaaataatatgaattaactttccagttctgtgacttttgaatgtgggtgctctttgctacttctaaacccccatcacttatcaacaggttggattccagcgagggaatcagaggctatttttagattgttcagtactcagctcaccacccataagaccatttctcctctgcgtgtggcctagttcttagatatactgtaatttctttcttccccaggacacttaagaaacagtttcattttcatgacaggcaagggcttcaggaagagtcgttccacagggtccctggaaatgaaacctgaatctgttcgtagctggggtggtctccgtgttaaattcagccactggcacgcccctggcagccacctggggggcaaacatggctgctgggtacaccacagaggaagtgcccaccactagacataaatcacagtgggcgagctctctgtcaacctcctccagaatggcaggatccaggttttctccaaaccacacgacgtgaggtcgcagcaagcccccgcagcctgcctcttcacacccttttcctgataaagctggacaaattggactcttgtaattctcagccacaactccacaagaggtacatcgagttttaaataagctaccatggatctccagaaggttcttggtgccagccttgcggtgcagctcatcgatgttctgggtgatgaccacgactcgccggccctgcttgcccagccgggtctcacactcggctatggcgcggtgcccggcgttgggctccttgctccccatgacctcccgccggtagtggtagaactcccacacccgggacgggttgtgggcaaaggccaggggagtcgccaggtcctgggcttgccattttctccaataacctccagctcctctgaaggtcggaacaccactttctgcactaacaccagctcctgagatgatgactatgtgctttgcttttgcaaaaaactttcgaaaatctgccatacttgaacttggccgagccattttcaggcaaatctggtttcgtgtggacgctggaggcttcaggccacaatatagctgggaaatcaatcgacttgggacaatctggagaggtcgcatcagggtttgtctgtagttctaatgcttgaggcgggctttagttatttctcccaaaatgaagatggttgtctccacggctgctttctaatatatttgaatctggagacatcaatataatacagacttctaatttgatccagaaaattattttcttcttctgtaggtttttatatgttagaaaacatttccatttactggggcagctcgcgcccccgaatacagtctcccacgccccgccccccggggtgcctccctcccagctctctgtacccacccaccatcccccacat

SEQ ID NO: 16762 - RNA, 2445 nt, Homo sapiens
  source 1..2445: mol_type = other RNA
taaggggtgtatggcagatgcatctgacagcaataacttaagaagtgagggttgccacgtggaggctgctgaggggagggtgctgagtgaaagtgctatgtaaactgcatgctttttataagtggttgcagttctgtccagcccgcggccactggaccaccctgtaaggttccccaaataaaccctatgtttccttcactagctccaggtctcttctttggcctcttgaacctggtgccatccctactgaagttaacagaggtctggcccaacctaagggcatcattttttaaagtcccatggaaaaaactcccagcagagttcagcatctgggaacggttggcaggccccacaggaaccacagcttctgcctttatgatgctgagaaacacttcactgttgacttcccccatctaagggggccagagctaaattttgggcagctgtgtttatcctgggggtccacatatttgcatcattctttcttctcatcgtgatgttctaccttgttggtactgttctcttccttctttgtgtgagttcctgttgtgagcttccccttgttcactgaggtaatgtagccaaacaaggttaaaaagcccccagtaagccgggtgcggtggctcatgcccgtaatctcagcactttgggaggccgaggcgggcagatcacctgaggtcgagagtttaagaccagcctgaccaacatggagaaaccccgtctctactaaaaatacaaaattagctgggtgtggtggtacatacctgtaatcccagctactcatgaggctgaggcaggagaatctcttgaacccgggaggcggaggttgctgtgagctgagatcgcaccactgcactccagcctgggcaacaagagtgaaactctgtctcaaaaaaaaaaaaaaaaagtccctaataaagccatatcgtggggtaatgtctttatacaataaattacctactgtagagtgtgattttattttccactaaaacttgtgcaaaaatcagaatagtagggtttttaccccttgacttctactttgcccagataacaaaaatataatcagaataactattttttttagacaatctaatttacaaaatttttccctcccaataaccaaccatacacatcaaagatacctcacgtttcagttcaaaccaaataatatgaattaactttccagttctgtgacttttgaatgtgggtgctctttgctacttctaaacccccatcacttatcaacaggttggattccagcgagggaatcagaggctatttttagattgttcagtactcagctcaccacccataagaccatttctcctctgcgtgtggcctagttcttagatatactgtaatttctttcttccccaggacacttaagaaacagtttcattttcatgacaggcaagggcttcaggaagagtcgttccacagggtccctggaaatgaaacctgaatctgttcgtagctggggtggtctccgtgttaaattcagccactggcacgcccctggcagccacctggggggcaaacatggctgctgggtacaccacagaggaagtgcccaccactagacataaatcacagtgggcgagctctctgtcaacctcctccagaatggcaggatccaggttttctccaaaccacacgacgtgaggtcgcagcaagcccccgcagcctgcctcttcacaccggggaagtttctcaactgggatgctggcatcttgagttccaggttctggagcacatggatctccagaaggttcttggtgccagccttgcggtgcagctcatcgatgttctgggtgatgaccacgactcgccggccctgcttgcccagccgggtctcacactcggctatggcgcggtgcccggcgttgggctccttgctccccatgacctcccgccggtagtggtagaactcccacacccgggacgggttgtgggcaaaggccaggggagtcgccaggtcctgggcttgccattttctccaataacctccagctcctctgaaggtcggaacaccactttctgcactaacaccagctcctgagatgatgactatgtgctttgcttttgcaaaaaactttcgaaaatctgccatacttgaacttggccgagccattttcaggcaaatctggtttcgtgtggacgctggaggcttcaggccacaatatagctgggaaatcaatcgacttgggacaatctggagaggtcgcatcagggtttgtctgtagttctaatgcttgaggcgggctttagttatttctcccaaaatgaagatggttgtctccacggctgctttctaatatatttgaatctggagacatcaatataatacagacttctaatttgatccagaaaattattttcttcttctgtaggtttttatatgttagaaaacatttccatttactggggcagctcgcgcccccgaat

SEQ ID NO: 16763 - RNA, 2540 nt, Homo sapiens
  source 1..2540: mol_type = other RNA
taaggggtgtatggcagatgcatctgacagcaataacttaagaagtgagggttgccacgtggaggctgctgaggggagggtgctgagtgaaagtgctatgtaaactgcatgctttttataagtggttgcagttctgtccagcccgcggccactggaccaccctgtaaggttccccaaataaaccctatgtttccttcactagctccaggtctcttctttggcctcttgaacctggtgccatccctactgaagttaacagaggtctggcccaacctaagggcatcattttttaaagtcccatggaaaaaactcccagcagagttcagcatctgggaacggttggcaggccccacaggaaccacagcttctgcctttatgatgctgagaaacacttcactgttgacttcccccatctaagggggccagagctaaattttgggcagctgtgtttatcctgggggtccacatatttgcatcattctttcttctcatcgtgatgttctaccttgttggtactgttctcttccttctttgtgtgagttcctgttgtgagcttccccttgttcactgaggtaatgtagccaaacaaggttaaaaagcccccagtaagccgggtgcggtggctcatgcccgtaatctcagcactttgggaggccgaggcgggcagatcacctgaggtcgagagtttaagaccagcctgaccaacatggagaaaccccgtctctactaaaaatacaaaattagctgggtgtggtggtacatacctgtaatcccagctactcatgaggctgaggcaggagaatctcttgaacccgggaggcggaggttgctgtgagctgagatcgcaccactgcactccagcctgggcaacaagagtgaaactctgtctcaaaaaaaaaaaaaaaaagtccctaataaagccatatcgtggggtaatgtctttatacaataaattacctactgtagagtgtgattttattttccactaaaacttgtgcaaaaatcagaatagtagggtttttaccccttgacttctactttgcccagataacaaaaatataatcagaataactattttttttagacaatctaatttacaaaatttttccctcccaataaccaaccatacacatcaaagatacctcacgtttcagttcaaaccaaataatatgaattaactttccagttctgtgacttttgaatgtgggtgctctttgctacttctaaacccccatcacttatcaacaggttggattccagcgagggaatcagaggctatttttagattgttcagtactcagctcaccacccataagaccatttctcctctgcgtgtggcctagttcttagatatactgtaatttctttcttccccaggacacttaagaaacagtttcattttcatgacaggcaagggcttcaggaagagtcgttccacagggtccctggaaatgaaacctgaatctgttcgtagctggggtggtctccgtgttaaattcagccactggcacgcccctggcagccacctggggggcaaacatggctgctgggtacaccacagaggaagtgcccaccactagacataaatcacagtgggcgagctctctgtcaacctcctccagaatggcaggatccaggttttctccaaaccacacgacgtgaggtcgcagcaagcccccgcagcctgcctcttcacaccggggaagtttctcaactgggatgctggcatcttgagttccaggttctggagcaccttttcctgataaagctggacaaattggactcttgtaattctcagccacaactccacaagaggtacatcgagttttaaataagctaccatggatctccagaaggttcttggtgccagccttgcggtgcagctcatcgatgttctgggtgatgaccacgactcgccggccctgcttgcccagccgggtctcacactcggctatggcgcggtgcccggcgttgggctccttgctccccatgacctcccgccggtagtggtagaactcccacacccgggacgggttgtgggcaaaggccaggggagtcgccaggtcctgaactcacatcccttccagagataggctgcttgtttttgtcaggtttgtcaaagatcagatggttgtagatgtgtagtgttatttctgaggcctctgttctgttccaccgtgaccgtcttaatttctctcagccttgtgttgaacttggccgagccattttcaggcaaatctggtttcgtgtggacgctggaggcttcaggccacaatatagctgggaaatcaatcgacttgggacaatctggagaggtcgcatcagggtttgtctgtagttctaatgcttgaggcgggctttagttatttctcccaaaatgaagatggttgtctccacggctgctttctaatatatttgaatctggagacatcaatataatacagacttctaatttgatccagaaaattattttcttcttctgtaggtttttatatgttagaaaacatttccatttactggggcagctcgcgcccccgaat

SEQ ID NO: 16764 - RNA, 2740 nt, Homo sapiens
  source 1..2740: mol_type = other RNA
taaggggtgtatggcagatgcatctgacagcaataacttaagaagtgagggttgccacgtggaggctgctgaggggagggtgctgagtgaaagtgctatgtaaactgcatgctttttataagtggttgcagttctgtccagcccgcggccactggaccaccctgtaaggttccccaaataaaccctatgtttccttcactagctccaggtctcttctttggcctcttgaacctggtgccatccctactgaagttaacagaggtctggcccaacctaagggcatcattttttaaagtcccatggaaaaaactcccagcagagttcagcatctgggaacggttggcaggccccacaggaaccacagcttctgcctttatgatgctgagaaacacttcactgttgacttcccccatctaagggggccagagctaaattttgggcagctgtgtttatcctgggggtccacatatttgcatcattctttcttctcatcgtgatgttctaccttgttggtactgttctcttccttctttgtgtgagttcctgttgtgagcttccccttgttcactgaggtaatgtagccaaacaaggttaaaaagcccccagtaagccgggtgcggtggctcatgcccgtaatctcagcactttgggaggccgaggcgggcagatcacctgaggtcgagagtttaagaccagcctgaccaacatggagaaaccccgtctctactaaaaatacaaaattagctgggtgtggtggtacatacctgtaatcccagctactcatgaggctgaggcaggagaatctcttgaacccgggaggcggaggttgctgtgagctgagatcgcaccactgcactccagcctgggcaacaagagtgaaactctgtctcaaaaaaaaaaaaaaaaagtccctaataaagccatatcgtggggtaatgtctttatacaataaattacctactgtagagtgtgattttattttccactaaaacttgtgcaaaaatcagaatagtagggtttttaccccttgacttctactttgcccagataacaaaaatataatcagaataactattttttttagacaatctaatttacaaaatttttccctcccaataaccaaccatacacatcaaagatacctcacgtttcagttcaaaccaaataatatgaattaactttccagttctgtgacttttgaatgtgggtgctctttgctacttctaaacccccatcacttatcaacaggttggattccagcgagggaatcagaggctatttttagattgttcagtactcagctcaccacccataagaccatttctcctctgcgtgtggcctagttcttagatatactgtaatttctttcttccccaggacacttaagaaacagtttcattttcatgacaggcaagggcttcaggaagagtcgttccacagggtccctggaaatgaaacctgaatctgttcgtagctggggtggtctccgtgttaaattcagccactggcacgcccctggcagccacctggggggcaaacatggctgctgggtacaccacagaggaagtgcccaccactagacataaatcacagtgggcgagctctctgtcaacctcctccagaatggcaggatccaggttttctccaaaccacacgacgtgaggtcgcagcaagcccccgcagcctgcctcttcacaccggggaagtttctcaactgggatgctggcatcttgagttccaggttctggagcaccttttcctgataaagctggacaaattggactcttgtaattctcagccacaactccacaagaggtacatcgagttttaaataagctaccatggatctccagaaggttcttggtgccagccttgcggtgcagctcatcgatgttctgggtgatgaccacgactcgccggccctgcttgcccagccgggtctcacactcggctatggcgcggtgcccggcgttgggctccttgctccccatgacctcccgccggtagtggtagaactcccacacccgggacgggttgtgggcaaaggccaggggagtcgccaggtcctgggcttgccattttctccaataacctccagctcctctgaaggtcggaacaccactttctgcactaacaccagctcctgagatgatgactatgtgctttgcttttgcaaaaaactttcgaaaatctgccatacctgaactcacatcccttccagagataggctgcttgtttttgtcaggtttgtcaaagatcagatggttgtagatgtgtagtgttatttctgaggcctctgttctgttccaccgtgaccgtcttaatttctctcagccttgtgttgaacttggccgagccattttcaggcaaatctggtttcgtgtggacgctggaggcttcaggccacaatatagctgggaaatcaatcgacttgggacaatctggagaggtcgcatcagggtttgtctgtagttctaatgcttgaggcgggctttagttatttctcccaaaatgaagatggttgtctccacggctgctttctaatatatttgaatctggagacatcaatataatacagacttctaatttgatccagaaaattattttcttcttctgtaggtttttatatgttagaaaacatttccatttactgcgggaggcgggcgcgccggctggagaggaggccgtggggcggagcggctcagcgttctgctcggctgcagcggcccctgccggagac

SEQ ID NO: 16765 - RNA, 2882 nt, Homo sapiens
  source 1..2882: mol_type = other RNA
taaggggtgtatggcagatgcatctgacagcaataacttaagaagtgagggttgccacgtggaggctgctgaggggagggtgctgagtgaaagtgctatgtaaactgcatgctttttataagtggttgcagttctgtccagcccgcggccactggaccaccctgtaaggttccccaaataaaccctatgtttccttcactagctccaggtctcttctttggcctcttgaacctggtgccatccctactgaagttaacagaggtctggcccaacctaagggcatcattttttaaagtcccatggaaaaaactcccagcagagttcagcatctgggaacggttggcaggccccacaggaaccacagcttctgcctttatgatgctgagaaacacttcactgttgacttcccccatctaagggggccagagctaaattttgggcagctgtgtttatcctgggggtccacatatttgcatcattctttcttctcatcgtgatgttctaccttgttggtactgttctcttccttctttgtgtgagttcctgttgtgagcttccccttgttcactgaggtaatgtagccaaacaaggttaaaaagcccccagtaagccgggtgcggtggctcatgcccgtaatctcagcactttgggaggccgaggcgggcagatcacctgaggtcgagagtttaagaccagcctgaccaacatggagaaaccccgtctctactaaaaatacaaaattagctgggtgtggtggtacatacctgtaatcccagctactcatgaggctgaggcaggagaatctcttgaacccgggaggcggaggttgctgtgagctgagatcgcaccactgcactccagcctgggcaacaagagtgaaactctgtctcaaaaaaaaaaaaaaaaagtccctaataaagccatatcgtggggtaatgtctttatacaataaattacctactgtagagtgtgattttattttccactaaaacttgtgcaaaaatcagaatagtagggtttttaccccttgacttctactttgcccagataacaaaaatataatcagaataactattttttttagacaatctaatttacaaaatttttccctcccaataaccaaccatacacatcaaagatacctcacgtttcagttcaaaccaaataatatgaattaactttccagttctgtgacttttgaatgtgggtgctctttgctacttctaaacccccatcacttatcaacaggttggattccagcgagggaatcagaggctatttttagattgttcagtactcagctcaccacccataagaccatttctcctctgcgtgtggcctagttcttagatatactgtaatttctttcttccccaggacacttaagaaacagtttcattttcatgacaggcaagggcttcaggaagagtcgttccacagggtccctggaaatgaaacctgaatctgttcgtagctggggtggtctccgtgttaaattcagccactggcacgcccctggcagccacctggggggcaaacatggctgctgggtacaccacagaggaagtgcccaccactagacataaatcacagtgggcgagctctctgtcaacctcctccagaatggcaggatccaggttttctccaaaccacacgacgtgaggtcgcagcaagcccccgcagcctgcctcttcacaccggggaagtttctcaactgggatgctggcatcttgagttccaggttctggagcaccttttcctgataaagctggacaaattggactcttgtaattctcagccacaactccacaagaggtacatcgagttttaaataagctaccatggatctccagaaggttcttggtgccagccttgcggtgcagctcatcgatgttctgggtgatgaccacgactcgccggccctgcttgcccagccgggtctcacactcggctatggcgcggtgcccggcgttgggctccttgctccccatgacctcccgccggtagtggtagaactcccacacccgggacgggttgtgggcaaaggccaggggagtcgccaggtcctgggcttgccattttctccaataacctccagctcctctgaaggtcggaacaccactttctgcactaacaccagctcctgagatgatgactatgtgctttgcttttgcaaaaaactttcgaaaatctgccatacctgaactcacatcccttccagagataggctgcttgtttttgtcaggtttgtcaaagatcagatggttgtagatgtgtagtgttatttctgaggcctctgttctgttccaccgtgaccgtcttaatttctctcagccttgtgttgaacttggccgagccattttcaggcaaatctggtttcgtgtggacgctggaggcttcaggccacaatatagctgggaaatcaatcgacttgggacaatctggagaggtcgcatcagggtttgtctgtagttctaatgcttgaggcgggctttagttatttctcccaaaatgaagatggttgtctccacggctgctttctaatatatttgaatctggagacatcaatataatacagacttctaatttgatccagaaaattattttcttcttctgtaggtttttatatgttagaaaacatttccatttactgctcgggtgggattactttccaaccccgtttccatccccctccctggtctccagccgcagcgacccccacgcagagcccggaagaccttgggccccgcacatgctgccggcccgctaagagctctgggtacccccggagcgccttccaggctttctcctagaggcgctgtgtcccgaccgcgctccggacctgagccacggctcacctggggcagctcgcgcccccgaat

SEQ ID NO: 16766 - RNA, 2676 nt, Homo sapiens
  source 1..2676: mol_type = other RNA
taaggggtgtatggcagatgcatctgacagcaataacttaagaagtgagggttgccacgtggaggctgctgaggggagggtgctgagtgaaagtgctatgtaaactgcatgctttttataagtggttgcagttctgtccagcccgcggccactggaccaccctgtaaggttccccaaataaaccctatgtttccttcactagctccaggtctcttctttggcctcttgaacctggtgccatccctactgaagttaacagaggtctggcccaacctaagggcatcattttttaaagtcccatggaaaaaactcccagcagagttcagcatctgggaacggttggcaggccccacaggaaccacagcttctgcctttatgatgctgagaaacacttcactgttgacttcccccatctaagggggccagagctaaattttgggcagctgtgtttatcctgggggtccacatatttgcatcattctttcttctcatcgtgatgttctaccttgttggtactgttctcttccttctttgtgtgagttcctgttgtgagcttccccttgttcactgaggtaatgtagccaaacaaggttaaaaagcccccagtaagccgggtgcggtggctcatgcccgtaatctcagcactttgggaggccgaggcgggcagatcacctgaggtcgagagtttaagaccagcctgaccaacatggagaaaccccgtctctactaaaaatacaaaattagctgggtgtggtggtacatacctgtaatcccagctactcatgaggctgaggcaggagaatctcttgaacccgggaggcggaggttgctgtgagctgagatcgcaccactgcactccagcctgggcaacaagagtgaaactctgtctcaaaaaaaaaaaaaaaaagtccctaataaagccatatcgtggggtaatgtctttatacaataaattacctactgtagagtgtgattttattttccactaaaacttgtgcaaaaatcagaatagtagggtttttaccccttgacttctactttgcccagataacaaaaatataatcagaataactattttttttagacaatctaatttacaaaatttttccctcccaataaccaaccatacacatcaaagatacctcacgtttcagttcaaaccaaataatatgaattaactttccagttctgtgacttttgaatgtgggtgctctttgctacttctaaacccccatcacttatcaacaggttggattccagcgagggaatcagaggctatttttagattgttcagtactcagctcaccacccataagaccatttctcctctgcgtgtggcctagttcttagatatactgtaatttctttcttccccaggacacttaagaaacagtttcattttcatgacaggcaagggcttcaggaagagtcgttccacagggtccctggaaatgaaacctgaatctgttcgtagctggggtggtctccgtgttaaattcagccactggcacgcccctggcagccacctggggggcaaacatggctgctgggtacaccacagaggaagtgcccaccactagacataaatcacagtgggcgagctctctgtcaacctcctccagaatggcaggatccaggttttctccaaaccacacgacgtgaggtcgcagcaagcccccgcagcctgcctcttcacaccggggaagtttctcaactgggatgctggcatcttgagttccaggttctggagcaccttttcctgataaagctggacaaattggactcttgtaattctcagccacaactccacaagaggtacatcgagttttaaataagctaccatggatctccagaaggttcttggtgccagccttgcggtgcagctcatcgatgttctgggtgatgaccacgactcgccggccctgcttgcccagccgggtctcacactcggctatggcgcggtgcccggcgttgggctccttgctccccatgacctcccgccggtagtggtagaactcccacacccgggacgggttgtgggcaaaggccaggggagtcgccaggtcctgggcttgccattttctccaataacctccagctcctctgaaggtcggaacaccactttctgcactaacaccagctcctgagatgatgactatgtgctttgcttttgcaaaaaactttcgaaaatctgccatacctgaactcacatcccttccagagataggctgcttgtttttgtcaggtttgtcaaagatcagatggttgtagatgtgtagtgttatttctgaggcctctgttctgttccaccgtgaccgtcttaatttctctcagccttgtgttgaacttggccgagccattttcaggcaaatctggtttcgtgtggacgctggaggcttcaggccacaatatagctgggaaatcaatcgacttgggacaatctggagaggtcgcatcagggtttgtctgtagttctaatgcttgaggcgggctttagttatttctcccaaaatgaagatggttgtctccacggctgctttctaatatatttgaatctggagacatcaatataatacagacttctaatttgatccagaaaattattttcttcttctgtaggtttttatatgttagaaaacatttccatttactggggcagctcgcgcccccgaatac

SEQ ID NO: 16767 - RNA, 2374 nt, Homo sapiens
  source 1..2374: mol_type = other RNA
taaggggtgtatggcagatgcatctgacagcaataacttaagaagtgagggttgccacgtggaggctgctgaggggagggtgctgagtgaaagtgctatgtaaactgcatgctttttataagtggttgcagttctgtccagcccgcggccactggaccaccctgtaaggttccccaaataaaccctatgtttccttcactagctccaggtctcttctttggcctcttgaacctggtgccatccctactgaagttaacagaggtctggcccaacctaagggcatcattttttaaagtcccatggaaaaaactcccagcagagttcagcatctgggaacggttggcaggccccacaggaaccacagcttctgcctttatgatgctgagaaacacttcactgttgacttcccccatctaagggggccagagctaaattttgggcagctgtgtttatcctgggggtccacatatttgcatcattctttcttctcatcgtgatgttctaccttgttggtactgttctcttccttctttgtgtgagttcctgttgtgagcttccccttgttcactgaggtaatgtagccaaacaaggttaaaaagcccccagtaagccgggtgcggtggctcatgcccgtaatctcagcactttgggaggccgaggcgggcagatcacctgaggtcgagagtttaagaccagcctgaccaacatggagaaaccccgtctctactaaaaatacaaaattagctgggtgtggtggtacatacctgtaatcccagctactcatgaggctgaggcaggagaatctcttgaacccgggaggcggaggttgctgtgagctgagatcgcaccactgcactccagcctgggcaacaagagtgaaactctgtctcaaaaaaaaaaaaaaaaagtccctaataaagccatatcgtggggtaatgtctttatacaataaattacctactgtagagtgtgattttattttccactaaaacttgtgcaaaaatcagaatagtagggtttttaccccttgacttctactttgcccagataacaaaaatataatcagaataactattttttttagacaatctaatttacaaaatttttccctcccaataaccaaccatacacatcaaagatacctcacgtttcagttcaaaccaaataatatgaattaactttccagttctgtgacttttgaatgtgggtgctctttgctacttctaaacccccatcacttatcaacaggttggattccagcgagggaatcagaggctatttttagattgttcagtactcagctcaccacccataagaccatttctcctctgcgtgtggcctagttcttagatatactgtaatttctttcttccccaggacacttaagaaacagtttcattttcatgacaggcaagggcttcaggaagagtcgttccacagggtccctggaaatgaaacctgaatctgttcgtagctggggtggtctccgtgttaaattcagccactggcacgcccctggcagccacctggggggcaaacatggctgctgggtacaccacagaggaagtgcccaccactagacataaatcacagtgggcgagctctctgtcaacctcctccagaatggcaggatccaggttttctccaaaccacacgacgtgaggtcgcagcaagcccccgcagcctgcctcttcacaccggggaagtttctcaactgggatgctggcatcttgagttccaggttctggagcaccttttcctgataaagctggacaaattggactcttgtaattctcagccacaactccacaagaggtacatcgagttttaaataagctaccatggatctccagaaggttcttggtgccagccttgcggtgcagctcatcgatgttctgggtgatgaccacgactcgccggccctgcttgcccagccgggtctcacactcggctatggcgcggtgcccggcgttgggctccttgctccccatgacctcccgccggtagtggtagaactcccacacccgggacgggttgtgggcaaaggccaggggagtcgccaggtcctgggcttgccattttctccaataacctccagctcctctgaaggtcggaacaccactttctgcactaacaccagctcctgagatgatgactatgtgctttgcttttgcaaaaaactttcgaaaatctgccatacttgaacttggccgagccattttcaggcaaatctggtttcgtgtggacgctggaggcttcaggccacaatatagctgggaaatcaatcgacttgggacaatctggagaggtcgcatcagggtttgtctgtagttctaatgcttgaggcgggctggggcagctcgcgcccccgaat

SEQ ID NO: 16768 - RNA, 2575 nt, Homo sapiens
  source 1..2575: mol_type = other RNA
taaggggtgtatggcagatgcatctgacagcaataacttaagaagtgagggttgccacgtggaggctgctgaggggagggtgctgagtgaaagtgctatgtaaactgcatgctttttataagtggttgcagttctgtccagcccgcggccactggaccaccctgtaaggttccccaaataaaccctatgtttccttcactagctccaggtctcttctttggcctcttgaacctggtgccatccctactgaagttaacagaggtctggcccaacctaagggcatcattttttaaagtcccatggaaaaaactcccagcagagttcagcatctgggaacggttggcaggccccacaggaaccacagcttctgcctttatgatgctgagaaacacttcactgttgacttcccccatctaagggggccagagctaaattttgggcagctgtgtttatcctgggggtccacatatttgcatcattctttcttctcatcgtgatgttctaccttgttggtactgttctcttccttctttgtgtgagttcctgttgtgagcttccccttgttcactgaggtaatgtagccaaacaaggttaaaaagcccccagtaagccgggtgcggtggctcatgcccgtaatctcagcactttgggaggccgaggcgggcagatcacctgaggtcgagagtttaagaccagcctgaccaacatggagaaaccccgtctctactaaaaatacaaaattagctgggtgtggtggtacatacctgtaatcccagctactcatgaggctgaggcaggagaatctcttgaacccgggaggcggaggttgctgtgagctgagatcgcaccactgcactccagcctgggcaacaagagtgaaactctgtctcaaaaaaaaaaaaaaaaagtccctaataaagccatatcgtggggtaatgtctttatacaataaattacctactgtagagtgtgattttattttccactaaaacttgtgcaaaaatcagaatagtagggtttttaccccttgacttctactttgcccagataacaaaaatataatcagaataactattttttttagacaatctaatttacaaaatttttccctcccaataaccaaccatacacatcaaagatacctcacgtttcagttcaaaccaaataatatgaattaactttccagttctgtgacttttgaatgtgggtgctctttgctacttctaaacccccatcacttatcaacaggttggattccagcgagggaatcagaggctatttttagattgttcagtactcagctcaccacccataagaccatttctcctctgcgtgtggcctagttcttagatatactgtaatttctttcttccccaggacacttaagaaacagtttcattttcatgacaggcaagggcttcaggaagagtcgttccacagggtccctggaaatgaaacctgaatctgttcgtagctggggtggtctccgtgttaaattcagccactggcacgcccctggcagccacctggggggcaaacatggctgctgggtacaccacagaggaagtgcccaccactagacataaatcacagtgggcgagctctctgtcaacctcctccagaatggcaggatccaggttttctccaaaccacacgacgtgaggtcgcagcaagcccccgcagcctgcctcttcacaccggggaagtttctcaactgggatgctggcatcttgagttccaggttctggagcaccttttcctgataaagctggacaaattggactcttgtaattctcagccacaactccacaagaggtacatcgagttttaaataagctaccatggatctccagaaggttcttggtgccagccttgcggtgcagctcatcgatgttctgggtgatgaccacgactcgccggccctgcttgcccagccgggtctcacactcggctatggcgcggtgcccggcgttgggctccttgctccccatgacctcccgccggtagtggtagaactcccacacccgggacgggttgtgggcaaaggccaggggagtcgccaggtcctgggcttgccattttctccaataacctccagctcctctgaaggtcggaacaccactttctgcactaacaccagctcctgagatgatgactatgtgctttgcttttgcaaaaaactttcgaaaatctgccatacttgaacttggccgagccattttcaggcaaatctggtttcgtgtggacgctggaggcttcaggccacaatatagctgggaaatcaatcgacttgggacaatctggagaggtcgcatcagggtttgtctgtagttctaatgcttgaggcgggctttagttatttctcccaaaatgaagatggttgtctccacggctgctttctaatatatttgaatctaacagattttttttaaaagcctgtatgttctctgtgaaaaaggggggcaccctaccaattccccggagcgccttccaggctttctcctagaggcgctgtgtcccgaccgcgctccggacctgagccacggctcacctggggcagctcgcgcccccgaat

SEQ ID NO: 16769 - RNA, 2608 nt, Homo sapiens
  source 1..2608: mol_type = other RNA
taaggggtgtatggcagatgcatctgacagcaataacttaagaagtgagggttgccacgtggaggctgctgaggggagggtgctgagtgaaagtgctatgtaaactgcatgctttttataagtggttgcagttctgtccagcccgcggccactggaccaccctgtaaggttccccaaataaaccctatgtttccttcactagctccaggtctcttctttggcctcttgaacctggtgccatccctactgaagttaacagaggtctggcccaacctaagggcatcattttttaaagtcccatggaaaaaactcccagcagagttcagcatctgggaacggttggcaggccccacaggaaccacagcttctgcctttatgatgctgagaaacacttcactgttgacttcccccatctaagggggccagagctaaattttgggcagctgtgtttatcctgggggtccacatatttgcatcattctttcttctcatcgtgatgttctaccttgttggtactgttctcttccttctttgtgtgagttcctgttgtgagcttccccttgttcactgaggtaatgtagccaaacaaggttaaaaagcccccagtaagccgggtgcggtggctcatgcccgtaatctcagcactttgggaggccgaggcgggcagatcacctgaggtcgagagtttaagaccagcctgaccaacatggagaaaccccgtctctactaaaaatacaaaattagctgggtgtggtggtacatacctgtaatcccagctactcatgaggctgaggcaggagaatctcttgaacccgggaggcggaggttgctgtgagctgagatcgcaccactgcactccagcctgggcaacaagagtgaaactctgtctcaaaaaaaaaaaaaaaaagtccctaataaagccatatcgtggggtaatgtctttatacaataaattacctactgtagagtgtgattttattttccactaaaacttgtgcaaaaatcagaatagtagggtttttaccccttgacttctactttgcccagataacaaaaatataatcagaataactattttttttagacaatctaatttacaaaatttttccctcccaataaccaaccatacacatcaaagatacctcacgtttcagttcaaaccaaataatatgaattaactttccagttctgtgacttttgaatgtgggtgctctttgctacttctaaacccccatcacttatcaacaggttggattccagcgagggaatcagaggctatttttagattgttcagtactcagctcaccacccataagaccatttctcctctgcgtgtggcctagttcttagatatactgtaatttctttcttccccaggacacttaagaaacagtttcattttcatgacaggcaagggcttcaggaagagtcgttccacagggtccctggaaatgaaacctgaatctgttcgtagctggggtggtctccgtgttaaattcagccactggcacgcccctggcagccacctggggggcaaacatggctgctgggtacaccacagaggaagtgcccaccactagacataaatcacagtgggcgagctctctgtcaacctcctccagaatggcaggatccaggttttctccaaaccacacgacgtgaggtcgcagcaagcccccgcagcctgcctcttcacaccggggaagtttctcaactgggatgctggcatcttgagttccaggttctggagcaccttttcctgataaagctggacaaattggactcttgtaattctcagccacaactccacaagaggtacatcgagttttaaataagctaccatggatctccagaaggttcttggtgccagccttgcggtgcagctcatcgatgttctgggtgatgaccacgactcgccggccctgcttgcccagccgggtctcacactcggctatggcgcggtgcccggcgttgggctccttgctccccatgacctcccgccggtagtggtagaactcccacacccgggacgggttgtgggcaaaggccaggggagtcgccaggtcctgggcttgccattttctccaataacctccagctcctctgaaggtcggaacaccactttctgcactaacaccagctcctgagatgatgactatgtgctttgcttttgcaaaaaactttcgaaaatctgccatacttgaacttggccgagccattttcaggcaaatctggtttcgtgtggacgctggaggcttcaggccacaatatagctgggaaatcaatcgacttgggacaatctggagaggtcgcatcagggtttgtctgtagttctaatgcttgaggcgggctttagttatttctcccaaaatgaagatggttgtctccacggctgctttctaatatatttgaatctggagacatcaatataatacagacttctaatttgatccagaaaattattttcttcttctgtaggtttttatatgttagaaaacatttccatttaccccggagcgccttccaggctttctcctagaggcgctgtgtcccgaccgcgctccggacctgagccacggctcacctggggcagctcgcgcccccgaat

SEQ ID NO: 16770 - RNA, 2663 nt, Homo sapiens
  source 1..2663: mol_type = other RNA
taaggggtgtatggcagatgcatctgacagcaataacttaagaagtgagggttgccacgtggaggctgctgaggggagggtgctgagtgaaagtgctatgtaaactgcatgctttttataagtggttgcagttctgtccagcccgcggccactggaccaccctgtaaggttccccaaataaaccctatgtttccttcactagctccaggtctcttctttggcctcttgaacctggtgccatccctactgaagttaacagaggtctggcccaacctaagggcatcattttttaaagtcccatggaaaaaactcccagcagagttcagcatctgggaacggttggcaggccccacaggaaccacagcttctgcctttatgatgctgagaaacacttcactgttgacttcccccatctaagggggccagagctaaattttgggcagctgtgtttatcctgggggtccacatatttgcatcattctttcttctcatcgtgatgttctaccttgttggtactgttctcttccttctttgtgtgagttcctgttgtgagcttccccttgttcactgaggtaatgtagccaaacaaggttaaaaagcccccagtaagccgggtgcggtggctcatgcccgtaatctcagcactttgggaggccgaggcgggcagatcacctgaggtcgagagtttaagaccagcctgaccaacatggagaaaccccgtctctactaaaaatacaaaattagctgggtgtggtggtacatacctgtaatcccagctactcatgaggctgaggcaggagaatctcttgaacccgggaggcggaggttgctgtgagctgagatcgcaccactgcactccagcctgggcaacaagagtgaaactctgtctcaaaaaaaaaaaaaaaaagtccctaataaagccatatcgtggggtaatgtctttatacaataaattacctactgtagagtgtgattttattttccactaaaacttgtgcaaaaatcagaatagtagggtttttaccccttgacttctactttgcccagataacaaaaatataatcagaataactattttttttagacaatctaatttacaaaatttttccctcccaataaccaaccatacacatcaaagatacctcacgtttcagttcaaaccaaataatatgaattaactttccagttctgtgacttttgaatgtgggtgctctttgctacttctaaacccccatcacttatcaacaggttggattccagcgagggaatcagaggctatttttagattgttcagtactcagctcaccacccataagaccatttctcctctgcgtgtggcctagttcttagatatactgtaatttctttcttccccaggacacttaagaaacagtttcattttcatgacaggcaagggcttcaggaagagtcgttccacagggtccctggaaatgaaacctgaatctgttcgtagctggggtggtctccgtgttaaattcagccactggcacgcccctggcagccacctggggggcaaacatggctgctgggtacaccacagaggaagtgcccaccactagacataaatcacagtgggcgagctctctgtcaacctcctccagaatggcaggatccaggttttctccaaaccacacgacgtgaggtcgcagcaagcccccgcagcctgcctcttcacaccggggaagtttctcaactgggatgctggcatcttgagttccaggttctggagcaccttttcctgataaagctggacaaattggactcttgtaattctcagccacaactccacaagaggtacatcgagttttaaataagctaccatggatctccagaaggttcttggtgccagccttgcggtgcagctcatcgatgttctgggtgatgaccacgactcgccggccctgcttgcccagccgggtctcacactcggctatggcgcggtgcccggcgttgggctccttgctccccatgacctcccgccggtagtggtagaactcccacacccgggacgggttgtgggcaaaggccaggggagtcgccaggtcctgggcttgccattttctccaataacctccagctcctctgaaggtcggaacaccactttctgcactaacaccagctcctgagatgatgactatgtgctttgcttttgcaaaaaactttcgaaaatctgccatacttgaacttggccgagccattttcaggcaaatctggtttcgtgtggacgctggaggcttcaggccacaatatagctgggaaatcaatcgacttgggacaatctggagaggtcgcatcagggtttgtctgtagttctaatgcttgaggcgggctttagttatttctcccaaaatgaagatggttgtctccacggctgctttctaatatatttgaatctggagacatcaatataatacagacttctaatttgatccagaaaattattttcttcttctgtaggtttttatatgttagaaaacatttccatttacgcggaccggtgccacctccgctcgcgagcccgcggcaggccctgggcggtgcgcgcagtcccgcgagagcagtgcttggtcgggacctcgaagccggagcccgagcgggagaggccgcggagaccccggcccggcgcaggcagagacgcacct

SEQ ID NO: 16771 - RNA, 2725 nt, Homo sapiens
  source 1..2725: mol_type = other RNA
taaggggtgtatggcagatgcatctgacagcaataacttaagaagtgagggttgccacgtggaggctgctgaggggagggtgctgagtgaaagtgctatgtaaactgcatgctttttataagtggttgcagttctgtccagcccgcggccactggaccaccctgtaaggttccccaaataaaccctatgtttccttcactagctccaggtctcttctttggcctcttgaacctggtgccatccctactgaagttaacagaggtctggcccaacctaagggcatcattttttaaagtcccatggaaaaaactcccagcagagttcagcatctgggaacggttggcaggccccacaggaaccacagcttctgcctttatgatgctgagaaacacttcactgttgacttcccccatctaagggggccagagctaaattttgggcagctgtgtttatcctgggggtccacatatttgcatcattctttcttctcatcgtgatgttctaccttgttggtactgttctcttccttctttgtgtgagttcctgttgtgagcttccccttgttcactgaggtaatgtagccaaacaaggttaaaaagcccccagtaagccgggtgcggtggctcatgcccgtaatctcagcactttgggaggccgaggcgggcagatcacctgaggtcgagagtttaagaccagcctgaccaacatggagaaaccccgtctctactaaaaatacaaaattagctgggtgtggtggtacatacctgtaatcccagctactcatgaggctgaggcaggagaatctcttgaacccgggaggcggaggttgctgtgagctgagatcgcaccactgcactccagcctgggcaacaagagtgaaactctgtctcaaaaaaaaaaaaaaaaagtccctaataaagccatatcgtggggtaatgtctttatacaataaattacctactgtagagtgtgattttattttccactaaaacttgtgcaaaaatcagaatagtagggtttttaccccttgacttctactttgcccagataacaaaaatataatcagaataactattttttttagacaatctaatttacaaaatttttccctcccaataaccaaccatacacatcaaagatacctcacgtttcagttcaaaccaaataatatgaattaactttccagttctgtgacttttgaatgtgggtgctctttgctacttctaaacccccatcacttatcaacaggttggattccagcgagggaatcagaggctatttttagattgttcagtactcagctcaccacccataagaccatttctcctctgcgtgtggcctagttcttagatatactgtaatttctttcttccccaggacacttaagaaacagtttcattttcatgacaggcaagggcttcaggaagagtcgttccacagggtccctggaaatgaaacctgaatctgttcgtagctggggtggtctccgtgttaaattcagccactggcacgcccctggcagccacctggggggcaaacatggctgctgggtacaccacagaggaagtgcccaccactagacataaatcacagtgggcgagctctctgtcaacctcctccagaatggcaggatccaggttttctccaaaccacacgacgtgaggtcgcagcaagcccccgcagcctgcctcttcacaccggggaagtttctcaactgggatgctggcatcttgagttccaggttctggagcaccttttcctgataaagctggacaaattggactcttgtaattctcagccacaactccacaagaggtacatcgagttttaaataagctaccatggatctccagaaggttcttggtgccagccttgcggtgcagctcatcgatgttctgggtgatgaccacgactcgccggccctgcttgcccagccgggtctcacactcggctatggcgcggtgcccggcgttgggctccttgctccccatgacctcccgccggtagtggtagaactcccacacccgggacgggttgtgggcaaaggccaggggagtcgccaggtcctgggcttgccattttctccaataacctccagctcctctgaaggtcggaacaccactttctgcactaacaccagctcctgagatgatgactatgtgctttgcttttgcaaaaaactttcgaaaatctgccatacttgaacttggccgagccattttcaggcaaatctggtttcgtgtggacgctggaggcttcaggccacaatatagctgggaaatcaatcgacttgggacaatctggagaggtcgcatcagggtttgtctgtagttctaatgcttgaggcgggctttagttatttctcccaaaatgaagatggttgtctccacggctgctttctaatatatttgaatctggagacatcaatataatacagacttctaatttgatccagaaaattattttcttcttctgtaggtttttatatgttagaaaacatttccatttactaacagattttttttaaaagcctgtatgttctctgtgaaaaaggggggcaccctaccaattcgcggaccggtgccacctccgctcgcgagcccgcggcaggccctgggcggtgcgcgcagtcccgcgagagcagtgcttggtcgggacctcgaagccggagcccgagcgggagaggccgcggagaccccggcccggcgcaggcagagacgcacct

SEQ ID NO: 16772 - RNA, 2604 nt, Homo sapiens
  source 1..2604: mol_type = other RNA
taaggggtgtatggcagatgcatctgacagcaataacttaagaagtgagggttgccacgtggaggctgctgaggggagggtgctgagtgaaagtgctatgtaaactgcatgctttttataagtggttgcagttctgtccagcccgcggccactggaccaccctgtaaggttccccaaataaaccctatgtttccttcactagctccaggtctcttctttggcctcttgaacctggtgccatccctactgaagttaacagaggtctggcccaacctaagggcatcattttttaaagtcccatggaaaaaactcccagcagagttcagcatctgggaacggttggcaggccccacaggaaccacagcttctgcctttatgatgctgagaaacacttcactgttgacttcccccatctaagggggccagagctaaattttgggcagctgtgtttatcctgggggtccacatatttgcatcattctttcttctcatcgtgatgttctaccttgttggtactgttctcttccttctttgtgtgagttcctgttgtgagcttccccttgttcactgaggtaatgtagccaaacaaggttaaaaagcccccagtaagccgggtgcggtggctcatgcccgtaatctcagcactttgggaggccgaggcgggcagatcacctgaggtcgagagtttaagaccagcctgaccaacatggagaaaccccgtctctactaaaaatacaaaattagctgggtgtggtggtacatacctgtaatcccagctactcatgaggctgaggcaggagaatctcttgaacccgggaggcggaggttgctgtgagctgagatcgcaccactgcactccagcctgggcaacaagagtgaaactctgtctcaaaaaaaaaaaaaaaaagtccctaataaagccatatcgtggggtaatgtctttatacaataaattacctactgtagagtgtgattttattttccactaaaacttgtgcaaaaatcagaatagtagggtttttaccccttgacttctactttgcccagataacaaaaatataatcagaataactattttttttagacaatctaatttacaaaatttttccctcccaataaccaaccatacacatcaaagatacctcacgtttcagttcaaaccaaataatatgaattaactttccagttctgtgacttttgaatgtgggtgctctttgctacttctaaacccccatcacttatcaacaggttggattccagcgagggaatcagaggctatttttagattgttcagtactcagctcaccacccataagaccatttctcctctgcgtgtggcctagttcttagatatactgtaatttctttcttccccaggacacttaagaaacagtttcattttcatgacaggcaagggcttcaggaagagtcgttccacagggtccctggaaatgaaacctgaatctgttcgtagctggggtggtctccgtgttaaattcagccactggcacgcccctggcagccacctggggggcaaacatggctgctgggtacaccacagaggaagtgcccaccactagacataaatcacagtgggcgagctctctgtcaacctcctccagaatggcaggatccaggttttctccaaaccacacgacgtgaggtcgcagcaagcccccgcagcctgcctcttcacaccggggaagtttctcaactgggatgctggcatcttgagttccaggttctggagcaccttttcctgataaagctggacaaattggactcttgtaattctcagccacaactccacaagaggtacatcgagttttaaataagctaccatggatctccagaaggttcttggtgccagccttgcggtgcagctcatcgatgttctgggtgatgaccacgactcgccggccctgcttgcccagccgggtctcacactcggctatggcgcggtgcccggcgttgggctccttgctccccatgacctcccgccggtagtggtagaactcccacacccgggacgggttgtgggcaaaggccaggggagtcgccaggtcctgggcttgccattttctccaataacctccagctcctctgaaggtcggaacaccactttctgcactaacaccagctcctgagatgatgactatgtgctttgcttttgcaaaaaactttcgaaaatctgccatacttgaacttggccgagccattttcaggcaaatctggtttcgtgtggacgctggaggcttcaggccacaatatagctgggaaatcaatcgacttgggacaatctggagaggtcgcatcagggtttgtctgtagttctaatgcttgaggcgggctttagttatttctcccaaaatgaagatggttgtctccacggctgctttctaatatatttgaatctggagacatcaatataatacagacttctaatttgatccagaaaattattttcttcttctgtaggtttttatatgttagaaaacatttccatttactaacagattttttttaaaagcctgtatgttctctgtgaaaaaggggggcaccctaccaattctgcgggaggcgggcgcgccggctggagaggag

SEQ ID NO: 16773 - RNA, 2549 nt, Homo sapiens
  source 1..2549: mol_type = other RNA
taaggggtgtatggcagatgcatctgacagcaataacttaagaagtgagggttgccacgtggaggctgctgaggggagggtgctgagtgaaagtgctatgtaaactgcatgctttttataagtggttgcagttctgtccagcccgcggccactggaccaccctgtaaggttccccaaataaaccctatgtttccttcactagctccaggtctcttctttggcctcttgaacctggtgccatccctactgaagttaacagaggtctggcccaacctaagggcatcattttttaaagtcccatggaaaaaactcccagcagagttcagcatctgggaacggttggcaggccccacaggaaccacagcttctgcctttatgatgctgagaaacacttcactgttgacttcccccatctaagggggccagagctaaattttgggcagctgtgtttatcctgggggtccacatatttgcatcattctttcttctcatcgtgatgttctaccttgttggtactgttctcttccttctttgtgtgagttcctgttgtgagcttccccttgttcactgaggtaatgtagccaaacaaggttaaaaagcccccagtaagccgggtgcggtggctcatgcccgtaatctcagcactttgggaggccgaggcgggcagatcacctgaggtcgagagtttaagaccagcctgaccaacatggagaaaccccgtctctactaaaaatacaaaattagctgggtgtggtggtacatacctgtaatcccagctactcatgaggctgaggcaggagaatctcttgaacccgggaggcggaggttgctgtgagctgagatcgcaccactgcactccagcctgggcaacaagagtgaaactctgtctcaaaaaaaaaaaaaaaaagtccctaataaagccatatcgtggggtaatgtctttatacaataaattacctactgtagagtgtgattttattttccactaaaacttgtgcaaaaatcagaatagtagggtttttaccccttgacttctactttgcccagataacaaaaatataatcagaataactattttttttagacaatctaatttacaaaatttttccctcccaataaccaaccatacacatcaaagatacctcacgtttcagttcaaaccaaataatatgaattaactttccagttctgtgacttttgaatgtgggtgctctttgctacttctaaacccccatcacttatcaacaggttggattccagcgagggaatcagaggctatttttagattgttcagtactcagctcaccacccataagaccatttctcctctgcgtgtggcctagttcttagatatactgtaatttctttcttccccaggacacttaagaaacagtttcattttcatgacaggcaagggcttcaggaagagtcgttccacagggtccctggaaatgaaacctgaatctgttcgtagctggggtggtctccgtgttaaattcagccactggcacgcccctggcagccacctggggggcaaacatggctgctgggtacaccacagaggaagtgcccaccactagacataaatcacagtgggcgagctctctgtcaacctcctccagaatggcaggatccaggttttctccaaaccacacgacgtgaggtcgcagcaagcccccgcagcctgcctcttcacaccggggaagtttctcaactgggatgctggcatcttgagttccaggttctggagcaccttttcctgataaagctggacaaattggactcttgtaattctcagccacaactccacaagaggtacatcgagttttaaataagctaccatggatctccagaaggttcttggtgccagccttgcggtgcagctcatcgatgttctgggtgatgaccacgactcgccggccctgcttgcccagccgggtctcacactcggctatggcgcggtgcccggcgttgggctccttgctccccatgacctcccgccggtagtggtagaactcccacacccgggacgggttgtgggcaaaggccaggggagtcgccaggtcctgggcttgccattttctccaataacctccagctcctctgaaggtcggaacaccactttctgcactaacaccagctcctgagatgatgactatgtgctttgcttttgcaaaaaactttcgaaaatctgccatacttgaacttggccgagccattttcaggcaaatctggtttcgtgtggacgctggaggcttcaggccacaatatagctgggaaatcaatcgacttgggacaatctggagaggtcgcatcagggtttgtctgtagttctaatgcttgaggcgggctttagttatttctcccaaaatgaagatggttgtctccacggctgctttctaatatatttgaatctggagacatcaatataatacagacttctaatttgatccagaaaattattttcttcttctgtaggtttttatatgttagaaaacatttccatttactgagccacggctcacctggggcagctcgcgcccccgaat

SEQ ID NO: 16774 - RNA, 2542 nt, Homo sapiens
  source 1..2542: mol_type = other RNA
taaggggtgtatggcagatgcatctgacagcaataacttaagaagtgagggttgccacgtggaggctgctgaggggagggtgctgagtgaaagtgctatgtaaactgcatgctttttataagtggttgcagttctgtccagcccgcggccactggaccaccctgtaaggttccccaaataaaccctatgtttccttcactagctccaggtctcttctttggcctcttgaacctggtgccatccctactgaagttaacagaggtctggcccaacctaagggcatcattttttaaagtcccatggaaaaaactcccagcagagttcagcatctgggaacggttggcaggccccacaggaaccacagcttctgcctttatgatgctgagaaacacttcactgttgacttcccccatctaagggggccagagctaaattttgggcagctgtgtttatcctgggggtccacatatttgcatcattctttcttctcatcgtgatgttctaccttgttggtactgttctcttccttctttgtgtgagttcctgttgtgagcttccccttgttcactgaggtaatgtagccaaacaaggttaaaaagcccccagtaagccgggtgcggtggctcatgcccgtaatctcagcactttgggaggccgaggcgggcagatcacctgaggtcgagagtttaagaccagcctgaccaacatggagaaaccccgtctctactaaaaatacaaaattagctgggtgtggtggtacatacctgtaatcccagctactcatgaggctgaggcaggagaatctcttgaacccgggaggcggaggttgctgtgagctgagatcgcaccactgcactccagcctgggcaacaagagtgaaactctgtctcaaaaaaaaaaaaaaaaagtccctaataaagccatatcgtggggtaatgtctttatacaataaattacctactgtagagtgtgattttattttccactaaaacttgtgcaaaaatcagaatagtagggtttttaccccttgacttctactttgcccagataacaaaaatataatcagaataactattttttttagacaatctaatttacaaaatttttccctcccaataaccaaccatacacatcaaagatacctcacgtttcagttcaaaccaaataatatgaattaactttccagttctgtgacttttgaatgtgggtgctctttgctacttctaaacccccatcacttatcaacaggttggattccagcgagggaatcagaggctatttttagattgttcagtactcagctcaccacccataagaccatttctcctctgcgtgtggcctagttcttagatatactgtaatttctttcttccccaggacacttaagaaacagtttcattttcatgacaggcaagggcttcaggaagagtcgttccacagggtccctggaaatgaaacctgaatctgttcgtagctggggtggtctccgtgttaaattcagccactggcacgcccctggcagccacctggggggcaaacatggctgctgggtacaccacagaggaagtgcccaccactagacataaatcacagtgggcgagctctctgtcaacctcctccagaatggcaggatccaggttttctccaaaccacacgacgtgaggtcgcagcaagcccccgcagcctgcctcttcacaccggggaagtttctcaactgggatgctggcatcttgagttccaggttctggagcaccttttcctgataaagctggacaaattggactcttgtaattctcagccacaactccacaagaggtacatcgagttttaaataagctaccatggatctccagaaggttcttggtgccagccttgcggtgcagctcatcgatgttctgggtgatgaccacgactcgccggccctgcttgcccagccgggtctcacactcggctatggcgcggtgcccggcgttgggctccttgctccccatgacctcccgccggtagtggtagaactcccacacccgggacgggttgtgggcaaaggccaggggagtcgccaggtcctgggcttgccattttctccaataacctccagctcctctgaaggtcggaacaccactttctgcactaacaccagctcctgagatgatgactatgtgctttgcttttgcaaaaaactttcgaaaatctgccatacttgaacttggccgagccattttcaggcaaatctggtttcgtgtggacgctggaggcttcaggccacaatatagctgggaaatcaatcgacttgggacaatctggagaggtcgcatcagggtttgtctgtagttctaatgcttgaggcgggctttagttatttctcccaaaatgaagatggttgtctccacggctgctttctaatatatttgaatctggagacatcaatataatacagacttctaatttgatccagaaaattattttcttcttctgtaggtttttatatgttagaaaacatttccatttactgcgggaggcgggcgcgccggctggagaggag

SEQ ID NO: 16775 - RNA, 2741 nt, Homo sapiens
  source 1..2741: mol_type = other RNA
taaggggtgtatggcagatgcatctgacagcaataacttaagaagtgagggttgccacgtggaggctgctgaggggagggtgctgagtgaaagtgctatgtaaactgcatgctttttataagtggttgcagttctgtccagcccgcggccactggaccaccctgtaaggttccccaaataaaccctatgtttccttcactagctccaggtctcttctttggcctcttgaacctggtgccatccctactgaagttaacagaggtctggcccaacctaagggcatcattttttaaagtcccatggaaaaaactcccagcagagttcagcatctgggaacggttggcaggccccacaggaaccacagcttctgcctttatgatgctgagaaacacttcactgttgacttcccccatctaagggggccagagctaaattttgggcagctgtgtttatcctgggggtccacatatttgcatcattctttcttctcatcgtgatgttctaccttgttggtactgttctcttccttctttgtgtgagttcctgttgtgagcttccccttgttcactgaggtaatgtagccaaacaaggttaaaaagcccccagtaagccgggtgcggtggctcatgcccgtaatctcagcactttgggaggccgaggcgggcagatcacctgaggtcgagagtttaagaccagcctgaccaacatggagaaaccccgtctctactaaaaatacaaaattagctgggtgtggtggtacatacctgtaatcccagctactcatgaggctgaggcaggagaatctcttgaacccgggaggcggaggttgctgtgagctgagatcgcaccactgcactccagcctgggcaacaagagtgaaactctgtctcaaaaaaaaaaaaaaaaagtccctaataaagccatatcgtggggtaatgtctttatacaataaattacctactgtagagtgtgattttattttccactaaaacttgtgcaaaaatcagaatagtagggtttttaccccttgacttctactttgcccagataacaaaaatataatcagaataactattttttttagacaatctaatttacaaaatttttccctcccaataaccaaccatacacatcaaagatacctcacgtttcagttcaaaccaaataatatgaattaactttccagttctgtgacttttgaatgtgggtgctctttgctacttctaaacccccatcacttatcaacaggttggattccagcgagggaatcagaggctatttttagattgttcagtactcagctcaccacccataagaccatttctcctctgcgtgtggcctagttcttagatatactgtaatttctttcttccccaggacacttaagaaacagtttcattttcatgacaggcaagggcttcaggaagagtcgttccacagggtccctggaaatgaaacctgaatctgttcgtagctggggtggtctccgtgttaaattcagccactggcacgcccctggcagccacctggggggcaaacatggctgctgggtacaccacagaggaagtgcccaccactagacataaatcacagtgggcgagctctctgtcaacctcctccagaatggcaggatccaggttttctccaaaccacacgacgtgaggtcgcagcaagcccccgcagcctgcctcttcacaccggggaagtttctcaactgggatgctggcatcttgagttccaggttctggagcaccttttcctgataaagctggacaaattggactcttgtaattctcagccacaactccacaagaggtacatcgagttttaaataagctaccatggatctccagaaggttcttggtgccagccttgcggtgcagctcatcgatgttctgggtgatgaccacgactcgccggccctgcttgcccagccgggtctcacactcggctatggcgcggtgcccggcgttgggctccttgctccccatgacctcccgccggtagtggtagaactcccacacccgggacgggttgtgggcaaaggccaggggagtcgccaggtcctgggcttgccattttctccaataacctccagctcctctgaaggtcggaacaccactttctgcactaacaccagctcctgagatgatgactatgtgctttgcttttgcaaaaaactttcgaaaatctgccatacttgaacttggccgagccattttcaggcaaatctggtttcgtgtggacgctggaggcttcaggccacaatatagctgggaaatcaatcgacttgggacaatctggagaggtcgcatcagggtttgtctgtagttctaatgcttgaggcgggctttagttatttctcccaaaatgaagatggttgtctccacggctgctttctaatatatttgaatctggagacatcaatataatacagacttctaatttgatccagaaaattattttcttcttctgtaggtttttatatgttagaaaacatttccatttactgctcgggtgggattactttccaaccccgtttccatccccctccctggtctccagccgcagcgacccccacgcagagcccggaagaccttgggccccgcacatgctgccggcccgctaagagctctgggtacccccggagcgccttccaggctttctcctagaggcgctgtgtcccgaccgcgctccggacctgagccacggctcacctggggcagctcgcgcccccgaat

SEQ ID NO: 16776 - RNA, 2533 nt, Homo sapiens
  source 1..2533: mol_type = other RNA
taaggggtgtatggcagatgcatctgacagcaataacttaagaagtgagggttgccacgtggaggctgctgaggggagggtgctgagtgaaagtgctatgtaaactgcatgctttttataagtggttgcagttctgtccagcccgcggccactggaccaccctgtaaggttccccaaataaaccctatgtttccttcactagctccaggtctcttctttggcctcttgaacctggtgccatccctactgaagttaacagaggtctggcccaacctaagggcatcattttttaaagtcccatggaaaaaactcccagcagagttcagcatctgggaacggttggcaggccccacaggaaccacagcttctgcctttatgatgctgagaaacacttcactgttgacttcccccatctaagggggccagagctaaattttgggcagctgtgtttatcctgggggtccacatatttgcatcattctttcttctcatcgtgatgttctaccttgttggtactgttctcttccttctttgtgtgagttcctgttgtgagcttccccttgttcactgaggtaatgtagccaaacaaggttaaaaagcccccagtaagccgggtgcggtggctcatgcccgtaatctcagcactttgggaggccgaggcgggcagatcacctgaggtcgagagtttaagaccagcctgaccaacatggagaaaccccgtctctactaaaaatacaaaattagctgggtgtggtggtacatacctgtaatcccagctactcatgaggctgaggcaggagaatctcttgaacccgggaggcggaggttgctgtgagctgagatcgcaccactgcactccagcctgggcaacaagagtgaaactctgtctcaaaaaaaaaaaaaaaaagtccctaataaagccatatcgtggggtaatgtctttatacaataaattacctactgtagagtgtgattttattttccactaaaacttgtgcaaaaatcagaatagtagggtttttaccccttgacttctactttgcccagataacaaaaatataatcagaataactattttttttagacaatctaatttacaaaatttttccctcccaataaccaaccatacacatcaaagatacctcacgtttcagttcaaaccaaataatatgaattaactttccagttctgtgacttttgaatgtgggtgctctttgctacttctaaacccccatcacttatcaacaggttggattccagcgagggaatcagaggctatttttagattgttcagtactcagctcaccacccataagaccatttctcctctgcgtgtggcctagttcttagatatactgtaatttctttcttccccaggacacttaagaaacagtttcattttcatgacaggcaagggcttcaggaagagtcgttccacagggtccctggaaatgaaacctgaatctgttcgtagctggggtggtctccgtgttaaattcagccactggcacgcccctggcagccacctggggggcaaacatggctgctgggtacaccacagaggaagtgcccaccactagacataaatcacagtgggcgagctctctgtcaacctcctccagaatggcaggatccaggttttctccaaaccacacgacgtgaggtcgcagcaagcccccgcagcctgcctcttcacaccggggaagtttctcaactgggatgctggcatcttgagttccaggttctggagcaccttttcctgataaagctggacaaattggactcttgtaattctcagccacaactccacaagaggtacatcgagttttaaataagctaccatggatctccagaaggttcttggtgccagccttgcggtgcagctcatcgatgttctgggtgatgaccacgactcgccggccctgcttgcccagccgggtctcacactcggctatggcgcggtgcccggcgttgggctccttgctccccatgacctcccgccggtagtggtagaactcccacacccgggacgggttgtgggcaaaggccaggggagtcgccaggtcctgggcttgccattttctccaataacctccagctcctctgaaggtcggaacaccactttctgcactaacaccagctcctgagatgatgactatgtgctttgcttttgcaaaaaactttcgaaaatctgccatacttgaacttggccgagccattttcaggcaaatctggtttcgtgtggacgctggaggcttcaggccacaatatagctgggaaatcaatcgacttgggacaatctggagaggtcgcatcagggtttgtctgtagttctaatgcttgaggcgggctttagttatttctcccaaaatgaagatggttgtctccacggctgctttctaatatatttgaatctggagacatcaatataatacagacttctaatttgatccagaaaattattttcttcttctgtaggtttttatatgttagaaaacatttccatttactggggcagctcgcgcccccgaat

SEQ ID NO: 16777 - RNA, 2653 nt, Homo sapiens
  source 1..2653: mol_type = other RNA
taaggggtgtatggcagatgcatctgacagcaataacttaagaagtgagggttgccacgtggaggctgctgaggggagggtgctgagtgaaagtgctatgtaaactgcatgctttttataagtggttgcagttctgtccagcccgcggccactggaccaccctgtaaggttccccaaataaaccctatgtttccttcactagctccaggtctcttctttggcctcttgaacctggtgccatccctactgaagttaacagaggtctggcccaacctaagggcatcattttttaaagtcccatggaaaaaactcccagcagagttcagcatctgggaacggttggcaggccccacaggaaccacagcttctgcctttatgatgctgagaaacacttcactgttgacttcccccatctaagggggccagagctaaattttgggcagctgtgtttatcctgggggtccacatatttgcatcattctttcttctcatcgtgatgttctaccttgttggtactgttctcttccttctttgtgtgagttcctgttgtgagcttccccttgttcactgaggtaatgtagccaaacaaggttaaaaagcccccagtaagccgggtgcggtggctcatgcccgtaatctcagcactttgggaggccgaggcgggcagatcacctgaggtcgagagtttaagaccagcctgaccaacatggagaaaccccgtctctactaaaaatacaaaattagctgggtgtggtggtacatacctgtaatcccagctactcatgaggctgaggcaggagaatctcttgaacccgggaggcggaggttgctgtgagctgagatcgcaccactgcactccagcctgggcaacaagagtgaaactctgtctcaaaaaaaaaaaaaaaaagtccctaataaagccatatcgtggggtaatgtctttatacaataaattacctactgtagagtgtgattttattttccactaaaacttgtgcaaaaatcagaatagtagggtttttaccccttgacttctactttgcccagataacaaaaatataatcagaataactattttttttagacaatctaatttacaaaatttttccctcccaataaccaaccatacacatcaaagatacctcacgtttcagttcaaaccaaataatatgaattaactttccagttctgtgacttttgaatgtgggtgctctttgctacttctaaacccccatcacttatcaacaggttggattccagcgagggaatcagaggctatttttagattgttcagtactcagctcaccacccataagaccatttctcctctgcgtgtggcctagttcttagatatactgtaatttctttcttccccaggacacttaagaaacagtttcattttcatgacaggcaagggcttcaggaagagtcgttccacagggtccctggaaatgaaacctgaatctgttcgtagctggggtggtctccgtgttaaattcagccactggcacgcccctggcagccacctggggggcaaacatggctgctgggtacaccacagaggaagtgcccaccactagacataaatcacagtgggcgagctctctgtcaacctcctccagaatggcaggatccaggttttctccaaaccacacgacgtgaggtcgcagcaagcccccgcagcctgcctcttcacaccggggaagtttctcaactgggatgctggcatcttgagttccaggttctggagcaccttttcctgataaagctggacaaattggactcttgtaattctcagccacaactccacaagaggtacatcgagttttaaataagctaccatggatctccagaaggttcttggtgccagccttgcggtgcagctcatcgatgttctgggtgatgaccacgactcgccggccctgcttgcccagccgggtctcacactcggctatggcgcggtgcccggcgttgggctccttgctccccatgacctcccgccggtagtggtagaactcccacacccgggacgggttgtgggcaaaggccaggggagtcgccaggtcctgggcttgccattttctccaataacctccagctcctctgaaggtcggaacaccactttctgcactaacaccagctcctgagatgatgactatgtgctttgcttttgcaaaaaactttcgaaaatctgccatacttgaacttggccgagccattttcaggcaaatctggtttcgtgtggacgctggaggcttcaggccacaatatagctgggaaatcaatcgacttgggacaatctggagaggtcgcatcagggtttgtctgtagttctaatgcttgaggcgggctttagttatttctcccaaaatgaagatggttgtctccacggctgctttctaatatatttgaatctggagacatcaatataatacagacttctaatttgatccagaaaattattttcttcttctgtaggtttttatatgttagaaaacatttccatttacttgggccccgcacatgctgccggcccgctaagagctctgggtacccccggagcgccttccaggctttctcctagaggcgctgtgtcccgaccgcgctccggacctgagccacggctcacctggggcagctcgcgcccccgaat

SEQ ID NO: 16778 - RNA, 2471 nt, Homo sapiens
  source 1..2471: mol_type = other RNA
taaggggtgtatggcagatgcatctgacagcaataacttaagaagtgagggttgccacgtggaggctgctgaggggagggtgctgagtgaaagtgctatgtaaactgcatgctttttataagtggttgcagttctgtccagcccgcggccactggaccaccctgtaaggttccccaaataaaccctatgtttccttcactagctccaggtctcttctttggcctcttgaacctggtgccatccctactgaagttaacagaggtctggcccaacctaagggcatcattttttaaagtcccatggaaaaaactcccagcagagttcagcatctgggaacggttggcaggccccacaggaaccacagcttctgcctttatgatgctgagaaacacttcactgttgacttcccccatctaagggggccagagctaaattttgggcagctgtgtttatcctgggggtccacatatttgcatcattctttcttctcatcgtgatgttctaccttgttggtactgttctcttccttctttgtgtgagttcctgttgtgagcttccccttgttcactgaggtaatgtagccaaacaaggttaaaaagcccccagtaagccgggtgcggtggctcatgcccgtaatctcagcactttgggaggccgaggcgggcagatcacctgaggtcgagagtttaagaccagcctgaccaacatggagaaaccccgtctctactaaaaatacaaaattagctgggtgtggtggtacatacctgtaatcccagctactcatgaggctgaggcaggagaatctcttgaacccgggaggcggaggttgctgtgagctgagatcgcaccactgcactccagcctgggcaacaagagtgaaactctgtctcaaaaaaaaaaaaaaaaagtccctaataaagccatatcgtggggtaatgtctttatacaataaattacctactgtagagtgtgattttattttccactaaaacttgtgcaaaaatcagaatagtagggtttttaccccttgacttctactttgcccagataacaaaaatataatcagaataactattttttttagacaatctaatttacaaaatttttccctcccaataaccaaccatacacatcaaagatacctcacgtttcagttcaaaccaaataatatgaattaactttccagttctgtgacttttgaatgtgggtgctctttgctacttctaaacccccatcacttatcaacaggttggattccagcgagggaatcagaggctatttttagattgttcagtactcagctcaccacccataagaccatttctcctctgcgtgtggcctagttcttagatatactgtaatttctttcttccccaggacacttaagaaacagtttcattttcatgacaggcaagggcttcaggaagagtcgttccacagggtccctggaaatgaaacctgaatctgttcgtagctggggtggtctccgtgttaaattcagccactggcacgcccctggcagccacctggggggcaaacatggctgctgggtacaccacagaggaagtgcccaccactagacataaatcacagtgggcgagctctctgtcaacctcctccagaatggcaggatccaggttttctccaaaccacacgacgtgaggtcgcagcaagcccccgcagcctgcctcttcacaccggggaagtttctcaactgggatgctggcatcttgagttccaggttctggagcaccttttcctgataaagctggacaaattggactcttgtaattctcagccacaactccacaagaggtacatcgagttttaaataagctaccatggatctccagaaggttcttggtgccagccttgcggtgcagctcatcgatgttctgggtgatgaccacgactcgccggccctgcttgcccagccgggtctcacactcggctatggcgcggtgcccggcgttgggctccttgctccccatgacctcccgccggtagtggtagaactcccacacccgggacgggttgtgggcaaaggccaggggagtcgccaggtcttgaacttggccgagccattttcaggcaaatctggtttcgtgtggacgctggaggcttcaggccacaatatagctgggaaatcaatcgacttgggacaatctggagaggtcgcatcagggtttgtctgtagttctaatgcttgaggcgggctttagttatttctcccaaaatgaagatggttgtctccacggctgctttctaatatatttgaatctggagacatcaatataatacagacttctaatttgatccagaaaattattttcttcttctgtaggtttttatatgttagaaaacatttccatttactggggcagctcgcgcccccgaatacagtctcccacgccccgccccccggggtgcctccctcccagctctctgtacccacccaccatcccccacat

SEQ ID NO: 16779 - RNA, 2529 nt, Homo sapiens
  source 1..2529: mol_type = other RNA
taaggggtgtatggcagatgcatctgacagcaataacttaagaagtgagggttgccacgtggaggctgctgaggggagggtgctgagtgaaagtgctatgtaaactgcatgctttttataagtggttgcagttctgtccagcccgcggccactggaccaccctgtaaggttccccaaataaaccctatgtttccttcactagctccaggtctcttctttggcctcttgaacctggtgccatccctactgaagttaacagaggtctggcccaacctaagggcatcattttttaaagtcccatggaaaaaactcccagcagagttcagcatctgggaacggttggcaggccccacaggaaccacagcttctgcctttatgatgctgagaaacacttcactgttgacttcccccatctaagggggccagagctaaattttgggcagctgtgtttatcctgggggtccacatatttgcatcattctttcttctcatcgtgatgttctaccttgttggtactgttctcttccttctttgtgtgagttcctgttgtgagcttccccttgttcactgaggtaatgtagccaaacaaggttaaaaagcccccagtaagccgggtgcggtggctcatgcccgtaatctcagcactttgggaggccgaggcgggcagatcacctgaggtcgagagtttaagaccagcctgaccaacatggagaaaccccgtctctactaaaaatacaaaattagctgggtgtggtggtacatacctgtaatcccagctactcatgaggctgaggcaggagaatctcttgaacccgggaggcggaggttgctgtgagctgagatcgcaccactgcactccagcctgggcaacaagagtgaaactctgtctcaaaaaaaaaaaaaaaaagtccctaataaagccatatcgtggggtaatgtctttatacaataaattacctactgtagagtgtgattttattttccactaaaacttgtgcaaaaatcagaatagtagggtttttaccccttgacttctactttgcccagataacaaaaatataatcagaataactattttttttagacaatctaatttacaaaatttttccctcccaataaccaaccatacacatcaaagatacctcacgtttcagttcaaaccaaataatatgaattaactttccagttctgtgacttttgaatgtgggtgctctttgctacttctaaacccccatcacttatcaacaggttggattccagcgagggaatcagaggctatttttagattgttcagtactcagctcaccacccataagaccatttctcctctgcgtgtggcctagttcttagatatactgtaatttctttcttccccaggacacttaagaaacagtttcattttcatgacaggcaagggcttcaggaagagtcgttccacagggtccctggaaatgaaacctgaatctgttcgtagctggggtggtctccgtgttaaattcagccactggcacgcccctggcagccacctggggggcaaacatggctgctgggtacaccacagaggaagtgcccaccggggaagtttctcaactgggatgctggcatcttgagttccaggttctggagcacatggatctccagaaggttcttggtgccagccttgcggtgcagctcatcgatgttctgggtgatgaccacgactcgccggccctgcttgcccagccgggtctcacactcggctatggcgcggtgcccggcgttgggctccttgctccccatgacctcccgccggtagtggtagaactcccacacccgggacgggttgtgggcaaaggccaggggagtcgccaggtcctgggcttgccattttctccaataacctccagctcctctgaaggtcggaacaccactttctgcactaacaccagctcctgagatgatgactatgtgctttgcttttgcaaaaaactttcgaaaatctgccatacttgaacttggccgagccattttcaggcaaatctggtttcgtgtggacgctggaggcttcaggccacaatatagctgggaaatcaatcgacttgggacaatctggagaggtcgcatcagggtttgtctgtagttctaatgcttgaggcgggctttagttatttctcccaaaatgaagatggttgtctccacggctgctttctaatatatttgaatctggagacatcaatataatacagacttctaatttgatccagaaaattattttcttcttctgtaggtttttatatgttagaaaacatttccatttactgctcgggtgggattactttccaaccccgtttccatccccctccctggtctccagccgcagcgacccccacgcagagcccggaagaccttgggccccgcacatgctgccggcccgctaagagctctgggtacccccggagcgccttccaggctttctcctagaggcgctgtgtcccgaccgcgctccggacctgagccacggctcacctggggcagctcgcgcccccgaat

SEQ ID NO: 16780 - RNA, 2321 nt, Homo sapiens
  source 1..2321: mol_type = other RNA
taaggggtgtatggcagatgcatctgacagcaataacttaagaagtgagggttgccacgtggaggctgctgaggggagggtgctgagtgaaagtgctatgtaaactgcatgctttttataagtggttgcagttctgtccagcccgcggccactggaccaccctgtaaggttccccaaataaaccctatgtttccttcactagctccaggtctcttctttggcctcttgaacctggtgccatccctactgaagttaacagaggtctggcccaacctaagggcatcattttttaaagtcccatggaaaaaactcccagcagagttcagcatctgggaacggttggcaggccccacaggaaccacagcttctgcctttatgatgctgagaaacacttcactgttgacttcccccatctaagggggccagagctaaattttgggcagctgtgtttatcctgggggtccacatatttgcatcattctttcttctcatcgtgatgttctaccttgttggtactgttctcttccttctttgtgtgagttcctgttgtgagcttccccttgttcactgaggtaatgtagccaaacaaggttaaaaagcccccagtaagccgggtgcggtggctcatgcccgtaatctcagcactttgggaggccgaggcgggcagatcacctgaggtcgagagtttaagaccagcctgaccaacatggagaaaccccgtctctactaaaaatacaaaattagctgggtgtggtggtacatacctgtaatcccagctactcatgaggctgaggcaggagaatctcttgaacccgggaggcggaggttgctgtgagctgagatcgcaccactgcactccagcctgggcaacaagagtgaaactctgtctcaaaaaaaaaaaaaaaaagtccctaataaagccatatcgtggggtaatgtctttatacaataaattacctactgtagagtgtgattttattttccactaaaacttgtgcaaaaatcagaatagtagggtttttaccccttgacttctactttgcccagataacaaaaatataatcagaataactattttttttagacaatctaatttacaaaatttttccctcccaataaccaaccatacacatcaaagatacctcacgtttcagttcaaaccaaataatatgaattaactttccagttctgtgacttttgaatgtgggtgctctttgctacttctaaacccccatcacttatcaacaggttggattccagcgagggaatcagaggctatttttagattgttcagtactcagctcaccacccataagaccatttctcctctgcgtgtggcctagttcttagatatactgtaatttctttcttccccaggacacttaagaaacagtttcattttcatgacaggcaagggcttcaggaagagtcgttccacagggtccctggaaatgaaacctgaatctgttcgtagctggggtggtctccgtgttaaattcagccactggcacgcccctggcagccacctggggggcaaacatggctgctgggtacaccacagaggaagtgcccaccggggaagtttctcaactgggatgctggcatcttgagttccaggttctggagcacatggatctccagaaggttcttggtgccagccttgcggtgcagctcatcgatgttctgggtgatgaccacgactcgccggccctgcttgcccagccgggtctcacactcggctatggcgcggtgcccggcgttgggctccttgctccccatgacctcccgccggtagtggtagaactcccacacccgggacgggttgtgggcaaaggccaggggagtcgccaggtcctgggcttgccattttctccaataacctccagctcctctgaaggtcggaacaccactttctgcactaacaccagctcctgagatgatgactatgtgctttgcttttgcaaaaaactttcgaaaatctgccatacttgaacttggccgagccattttcaggcaaatctggtttcgtgtggacgctggaggcttcaggccacaatatagctgggaaatcaatcgacttgggacaatctggagaggtcgcatcagggtttgtctgtagttctaatgcttgaggcgggctttagttatttctcccaaaatgaagatggttgtctccacggctgctttctaatatatttgaatctggagacatcaatataatacagacttctaatttgatccagaaaattattttcttcttctgtaggtttttatatgttagaaaacatttccatttactggggcagctcgcgcccccgaat

SEQ ID NO: 16781 - RNA, 2187 nt, Homo sapiens
  source 1..2187: mol_type = other RNA
taaggggtgtatggcagatgcatctgacagcaataacttaagaagtgagggttgccacgtggaggctgctgaggggagggtgctgagtgaaagtgctatgtaaactgcatgctttttataagtggttgcagttctgtccagcccgcggccactggaccaccctgtaaggttccccaaataaaccctatgtttccttcactagctccaggtctcttctttggcctcttgaacctggtgccatccctactgaagttaacagaggtctggcccaacctaagggcatcattttttaaagtcccatggaaaaaactcccagcagagttcagcatctgggaacggttggcaggccccacaggaaccacagcttctgcctttatgatgctgagaaacacttcactgttgacttcccccatctaagggggccagagctaaattttgggcagctgtgtttatcctgggggtccacatatttgcatcattctttcttctcatcgtgatgttctaccttgttggtactgttctcttccttctttgtgtgagttcctgttgtgagcttccccttgttcactgaggtaatgtagccaaacaaggttaaaaagcccccagtaagccgggtgcggtggctcatgcccgtaatctcagcactttgggaggccgaggcgggcagatcacctgaggtcgagagtttaagaccagcctgaccaacatggagaaaccccgtctctactaaaaatacaaaattagctgggtgtggtggtacatacctgtaatcccagctactcatgaggctgaggcaggagaatctcttgaacccgggaggcggaggttgctgtgagctgagatcgcaccactgcactccagcctgggcaacaagagtgaaactctgtctcaaaaaaaaaaaaaaaaagtccctaataaagccatatcgtggggtaatgtctttatacaataaattacctactgtagagtgtgattttattttccactaaaacttgtgcaaaaatcagaatagtagggtttttaccccttgacttctactttgcccagataacaaaaatataatcagaataactattttttttagacaatctaatttacaaaatttttccctcccaataaccaaccatacacatcaaagatacctcacgtttcagttcaaaccaaataatatgaattaactttccagttctgtgacttttgaatgtgggtgctctttgctacttctaaacccccatcacttatcaacaggttggattccagcgagggaatcagaggctatttttagattgttcagtactcagctcaccacccataagaccatttctcctctgcgtgtggcctagttcttagatatactgtaatttctttcttccccaggacacttaagaaacagtttcattttcatgacaggcaagggcttcaggaagagtcgttccacagggtccctggaaatgaaacctgaatctgttcgtagctggggtggtctccgtgttaaattcagccactggcacgcccctggcagccacctggggggcaaacatggctgctgggtacaccacagaggaagtgcccaccggggaagtttctcaactgggatgctggcatcttgagttccaggttctggagcacatggatctccagaaggttcttggtgccagccttgcggtgcagctcatcgatgttctgggtgatgaccacgactcgccggccctgcttgcccagccgggtctcacactcggctatggcgcggtgcccggcgttgggctccttgctccccatgacctcccgccggtagtggtagaactcccacacccgggacgggttgtgggcaaaggccaggggagtcgccaggtcttgaacttggccgagccattttcaggcaaatctggtttcgtgtggacgctggaggcttcaggccacaatatagctgggaaatcaatcgacttgggacaatctggagaggtcgcatcagggtttgtctgtagttctaatgcttgaggcgggctttagttatttctcccaaaatgaagatggttgtctccacggctgctttctaatatatttgaatctggagacatcaatataatacagacttctaatttgatccagaaaattattttcttcttctgtaggtttttatatgttagaaaacatttccatttactggggcagctcgcgcccccgaat

SEQ ID NO: 16782 - RNA, 2418 nt, Homo sapiens
  source 1..2418: mol_type = other RNA
taaggggtgtatggcagatgcatctgacagcaataacttaagaagtgagggttgccacgtggaggctgctgaggggagggtgctgagtgaaagtgctatgtaaactgcatgctttttataagtggttgcagttctgtccagcccgcggccactggaccaccctgtaaggttccccaaataaaccctatgtttccttcactagctccaggtctcttctttggcctcttgaacctggtgccatccctactgaagttaacagaggtctggcccaacctaagggcatcattttttaaagtcccatggaaaaaactcccagcagagttcagcatctgggaacggttggcaggccccacaggaaccacagcttctgcctttatgatgctgagaaacacttcactgttgacttcccccatctaagggggccagagctaaattttgggcagctgtgtttatcctgggggtccacatatttgcatcattctttcttctcatcgtgatgttctaccttgttggtactgttctcttccttctttgtgtgagttcctgttgtgagcttccccttgttcactgaggtaatgtagccaaacaaggttaaaaagcccccagtaagccgggtgcggtggctcatgcccgtaatctcagcactttgggaggccgaggcgggcagatcacctgaggtcgagagtttaagaccagcctgaccaacatggagaaaccccgtctctactaaaaatacaaaattagctgggtgtggtggtacatacctgtaatcccagctactcatgaggctgaggcaggagaatctcttgaacccgggaggcggaggttgctgtgagctgagatcgcaccactgcactccagcctgggcaacaagagtgaaactctgtctcaaaaaaaaaaaaaaaaagtccctaataaagccatatcgtggggtaatgtctttatacaataaattacctactgtagagtgtgattttattttccactaaaacttgtgcaaaaatcagaatagtagggtttttaccccttgacttctactttgcccagataacaaaaatataatcagaataactattttttttagacaatctaatttacaaaatttttccctcccaataaccaaccatacacatcaaagatacctcacgtttcagttcaaaccaaataatatgaattaactttccagttctgtgacttttgaatgtgggtgctctttgctacttctaaacccccatcacttatcaacaggttggattccagcgagggaatcagaggctatttttagattgttcagtactcagctcaccacccataagaccatttctcctctgcgtgtggcctagttcttagatatactgtaatttctttcttccccaggacacttaagaaacagtttcattttcatgacaggcaagggcttcaggaagagtcgttccacagggtccctggaaatgaaacctgaatctgttcgtagctggggtggtctccgtgttaaattcagccactggcacgcccctggcagccacctggggggcaaacatggctgctgggtacaccacagaggaagtgcccaccggggaagtttctcaactgggatgctggcatcttgagttccaggttctggagcaccttttcctgataaagctggacaaattggactcttgtaattctcagccacaactccacaagaggtacatcgagttttaaataagctaccatggatctccagaaggttcttggtgccagccttgcggtgcagctcatcgatgttctgggtgatgaccacgactcgccggccctgcttgcccagccgggtctcacactcggctatggcgcggtgcccggcgttgggctccttgctccccatgacctcccgccggtagtggtagaactcccacacccgggacgggttgtgggcaaaggccaggggagtcgccaggtcctgggcttgccattttctccaataacctccagctcctctgaaggtcggaacaccactttctgcactaacaccagctcctgagatgatgactatgtgctttgcttttgcaaaaaactttcgaaaatctgccatacttgaacttggccgagccattttcaggcaaatctggtttcgtgtggacgctggaggcttcaggccacaatatagctgggaaatcaatcgacttgggacaatctggagaggtcgcatcagggtttgtctgtagttctaatgcttgaggcgggctttagttatttctcccaaaatgaagatggttgtctccacggctgctttctaatatatttgaatctggagacatcaatataatacagacttctaatttgatccagaaaattattttcttcttctgtaggtttttatatgttagaaaacatttccatttactgcgggaggcgggcgcgccggctggagaggag

SEQ ID NO: 16783 - RNA, 2409 nt, Homo sapiens
  source 1..2409: mol_type = other RNA
taaggggtgtatggcagatgcatctgacagcaataacttaagaagtgagggttgccacgtggaggctgctgaggggagggtgctgagtgaaagtgctatgtaaactgcatgctttttataagtggttgcagttctgtccagcccgcggccactggaccaccctgtaaggttccccaaataaaccctatgtttccttcactagctccaggtctcttctttggcctcttgaacctggtgccatccctactgaagttaacagaggtctggcccaacctaagggcatcattttttaaagtcccatggaaaaaactcccagcagagttcagcatctgggaacggttggcaggccccacaggaaccacagcttctgcctttatgatgctgagaaacacttcactgttgacttcccccatctaagggggccagagctaaattttgggcagctgtgtttatcctgggggtccacatatttgcatcattctttcttctcatcgtgatgttctaccttgttggtactgttctcttccttctttgtgtgagttcctgttgtgagcttccccttgttcactgaggtaatgtagccaaacaaggttaaaaagcccccagtaagccgggtgcggtggctcatgcccgtaatctcagcactttgggaggccgaggcgggcagatcacctgaggtcgagagtttaagaccagcctgaccaacatggagaaaccccgtctctactaaaaatacaaaattagctgggtgtggtggtacatacctgtaatcccagctactcatgaggctgaggcaggagaatctcttgaacccgggaggcggaggttgctgtgagctgagatcgcaccactgcactccagcctgggcaacaagagtgaaactctgtctcaaaaaaaaaaaaaaaaagtccctaataaagccatatcgtggggtaatgtctttatacaataaattacctactgtagagtgtgattttattttccactaaaacttgtgcaaaaatcagaatagtagggtttttaccccttgacttctactttgcccagataacaaaaatataatcagaataactattttttttagacaatctaatttacaaaatttttccctcccaataaccaaccatacacatcaaagatacctcacgtttcagttcaaaccaaataatatgaattaactttccagttctgtgacttttgaatgtgggtgctctttgctacttctaaacccccatcacttatcaacaggttggattccagcgagggaatcagaggctatttttagattgttcagtactcagctcaccacccataagaccatttctcctctgcgtgtggcctagttcttagatatactgtaatttctttcttccccaggacacttaagaaacagtttcattttcatgacaggcaagggcttcaggaagagtcgttccacagggtccctggaaatgaaacctgaatctgttcgtagctggggtggtctccgtgttaaattcagccactggcacgcccctggcagccacctggggggcaaacatggctgctgggtacaccacagaggaagtgcccaccggggaagtttctcaactgggatgctggcatcttgagttccaggttctggagcaccttttcctgataaagctggacaaattggactcttgtaattctcagccacaactccacaagaggtacatcgagttttaaataagctaccatggatctccagaaggttcttggtgccagccttgcggtgcagctcatcgatgttctgggtgatgaccacgactcgccggccctgcttgcccagccgggtctcacactcggctatggcgcggtgcccggcgttgggctccttgctccccatgacctcccgccggtagtggtagaactcccacacccgggacgggttgtgggcaaaggccaggggagtcgccaggtcctgggcttgccattttctccaataacctccagctcctctgaaggtcggaacaccactttctgcactaacaccagctcctgagatgatgactatgtgctttgcttttgcaaaaaactttcgaaaatctgccatacttgaacttggccgagccattttcaggcaaatctggtttcgtgtggacgctggaggcttcaggccacaatatagctgggaaatcaatcgacttgggacaatctggagaggtcgcatcagggtttgtctgtagttctaatgcttgaggcgggctttagttatttctcccaaaatgaagatggttgtctccacggctgctttctaatatatttgaatctggagacatcaatataatacagacttctaatttgatccagaaaattattttcttcttctgtaggtttttatatgttagaaaacatttccatttactggggcagctcgcgcccccgaat

SEQ ID NO: 16784 - RNA, 1961 nt, Homo sapiens
  source 1..1961: mol_type = other RNA
taaggggtgtatggcagatgcatctgacagcaataacttaagaagtgagggttgccacgtggaggctgctgaggggagggtgctgagtgaaagtgctatgtaaactgcatgctttttataagtggttgcagttctgtccagcccgcggccactggaccaccctgtaaggttccccaaataaaccctatgtttccttcactagctccaggtctcttctttggcctcttgaacctggtgccatccctactgaagttaacagaggtctggcccaacctaagggcatcattttttaaagtcccatggaaaaaactcccagcagagttcagcatctgggaacggttggcaggccccacaggaaccacagcttctgcctttatgatgctgagaaacacttcactgttgacttcccccatctaagggggccagagctaaattttgggcagctgtgtttatcctgggggtccacatatttgcatcattctttcttctcatcgtgatgttctaccttgttggtactgttctcttccttctttgtgtgagttcctgttgtgagcttccccttgttcactgaggtaatgtagccaaacaaggttaaaaagcccccagtaagccgggtgcggtggctcatgcccgtaatctcagcactttgggaggccgaggcgggcagatcacctgaggtcgagagtttaagaccagcctgaccaacatggagaaaccccgtctctactaaaaatacaaaattagctgggtgtggtggtacatacctgtaatcccagctactcatgaggctgaggcaggagaatctcttgaacccgggaggcggaggttgctgtgagctgagatcgcaccactgcactccagcctgggcaacaagagtgaaactctgtctcaaaaaaaaaaaaaaaaagtccctaataaagccatatcgtggggtaatgtctttatacaataaattacctactgtagagtgtgattttattttccactaaaacttgtgcaaaaatcagaatagtagggtttttaccccttgacttctactttgcccagataacaaaaatataatcagaataactattttttttagacaatctaatttacaaaatttttccctcccaataaccaaccatacacatcaaagatacctcacgtttcagttcaaaccaaataatatgaattaactttccagttctgtgacttttgaatgtgggtgctctttgctacttctaaacccccatcacttatcaacaggttggattccagcgagggaatcagaggctatttttagattgttcagtactcagctcaccacccataagaccatttctcctctgcgtgtggcctagttcttagatatactgtaatttctttcttccccaggacacttaagaaacagtttcattttcatgacaggcaagggcttcaggaagagtcgttccacagggtccctggaaatgaaacctgaatctgttcgtagctggggtggtctccgtgttaaattcagccactggcacgcccctggcagccacctggggggcaaacatggctgctgggtacaccacagaggaagtgcccaccggggaagtttctcaactgggatgctggcatcttgagttccaggttctggagcattgaacttggccgagccattttcaggcaaatctggtttcgtgtggacgctggaggcttcaggccacaatatagctgggaaatcaatcgacttgggacaatctggagaggtcgcatcagggtttgtctgtagttctaatgcttgaggcgggctttagttatttctcccaaaatgaagatggttgtctccacggctgctttctaatatatttgaatctggagacatcaatataatacagacttctaatttgatccagaaaattattttcttcttctgtaggtttttatatgttagaaaacatttccatttactggggcagctcgcgcccccgaat

SEQ ID NO: 16785 - RNA, 5851 nt, Homo sapiens
  source 1..5851: mol_type = other RNA
taagtgcttccatgtttcagtggggacggccccaggaataaatctgccatggaaacatccagtatactgtgggtctctttcggagataaattgggtaataggagtttggaatcccaaaagggcagctctgagaggaagcagggtactccctttctccagggggtcctcgcatgcagcagagttctcaaacacctttagtttaggcccctcttaacctggtaagtggagcagaccttgtcctcatacatttttaaagggtttcagtcacacacttgctgaaatccatttgtggatttctgggaccatgatgccagagaagaggatgtgggctcagccataactaagaaggaactccgtagtaatgtccagatggggaagaggactcgagttctgagacttcaaagtgctgcccatttgtggcaaacacttcattgagaaatggcttctgtggatgcagtctaagcctggggtgcttattttaggcaactatggtatatacactcacttttatatacacatttctcatttgtcagatttcccacggtgaactggcaactcctctctgggtgaaatccaaacgtggtggaagacagattcctggttctgggccaggtcctgtcagtttctgatcattacctggttttctatttccaactccatttaggtgactgagtctccacacagagctcaggttgagctttagacacaaatctcatctggtcattcattatatgatttgtatcctccagtggcttctgcctttttgaaaagtccaaattacctactcttttctggtctcctattctgcaaattaaatcttcataagtgattatactttccacatatggaatggagggtggtagaaagctgtcatgtcggtctctcccattccgccactcctctgccttctgtgtgactgcatagggaaggacagtcaggatacccttctccccagcagagtagttggcccggtgttgaaaacttgacccaattaaaagctagtgagagagcaaggcctaaatatacccaggcctcaggatctagccatgggtaagtcactcctggacttatatgagctaatattattattatttaaactaatttgaagtccgtttctaaactttccactgaaataaacctagaactcagaccatattgaactaacctgcttatgataggtgtggaatctgtttataaggctttgaaaataactatgtttacatctttcaactgaacaggacataagtcgatggcatgattcatgatatccactctagcatatgtagcttgactccactgaatccactccccttcctctgatacgtcttctttaatacatcagtggcactatttacagcaaggatggtttcaatggaggttgctttaatattacatttcccttccttcaagagtctaatgccaactgtaacaggatttctcatcttttttcctatactcagagagcaaactgggccatttaaatcacccagttaatgtaccagttgctgttgaggagcagatggaggtctgcattagactccaccagaatctgtgctccagaaggcacagcctcaggaccagaggagctgagaacaccttgaggaccagacccttattcacaaaataaggagctgggtactaggcgaggaagttatttgactcagagcatcacggagtcaggtgaagaagacacctttgccccattccacaacactgctcctccaggacatcatgcagctcccacacaaggaacaacagccagatcctctggatgtcctataaattagttgaatcagaaactgagtaatatcagtgtgtcattataggtcatttagaaatagctttagtttcatagtaataataagctctgagctatatgacatattgctctaaactgtacagaaactcaactaacttgcagtcttttcttaggagtataacgtaggcttctggttaaatgtagcagattgactacacacttctcacctttcctttccaacaatgactaaaatgatagcaaataaaataaaaattaaagaaatagctaagggcaagagactaggagggaagatagcagaggagtgatttcaacaaattttggaaagacagaatagacagaatgatgcccaatttaacttcctcaactctgcgatagcctaaagaacctacggaggagataccaagaaaaataatttactctcatagaaacccagagaggctcaggtttggagagactgtataccacaaaaaacaggagtgagacatgaggctggaaactttagaaactagttgtaagtttatttagagagagattggacctccaggtctctgccttaacccttcacacatacaggactactgtctctcaccttgaccaccttccctaaagaacagagaactctgtgatatgaagaccacagacctcagttactacaggctttgactgaaatcaaaaaaggtattacatgaaagcatgtaatctgagccaggggtctccactgttcctttccttctccaaagtttcattctgccaaatgttggaagccaggccaacatctccaaagtagactagacaagtcttctctggaaaaactgcaaagacattcagattgacaaacacttggctccaaagcccacctgttggctaatccagctattcccatagagcttcaaatcagattttttacattcttttaggaaaaaaacaggtggccatatattcaaggaactaatccagcagaatagagaacgaccaaatcaaacaacagtataaaatgaacaccctccttctcataaaccacactgtttttcattgcttctaactccttactggtgctaacctaatcccacatcataggccatctttggcagtagaccaatactgcaaggtatacccagattcattagaaatattctggacttaagcaagatattaaattctttcagaataccatttgagttcatgtgtgtcaggagagtaatagctaggctgaaagactaaacttggagaaaaagccttcagtgatatgttacaaggcattcattctagtatattcacatcattggtaagtatgtcaatggtataattctcaaacttctggatgacaccactttaggaggaggaacagccaatatagaagctgagagaaccagaaccccatccaaagagaatctgaagagattcagataataaaggacaaaattaactggaaaaaaaattaagtcttacattcacatttaaaaacaactacgcaaaacagagatatgaattagtaagagttaattattagttttttttttaatccctcaagaatctgggtttcctatacattcagtgactcatcaatgaagcagctgcccaaaaaactaatgccttcttagacaacagcaggagaggcagagtgcccagggcattgcacttcaagagggttatgaacaaggaacatgaccacacgggggtaaccagatggacacagttcaagaccatgcaccacagagaaatgtgcttcccatctcgggtacttcagagagccattcccttccatctcaccaaaaggaacaaaaaactgtgtactgtggaaatcgagaaagcaaagccgtgactttaccaaaagtaacaggagtcagtcaggcaagacccggacaagctgggtgataggagccagtggtggtgagagtttcctctcctcagtgagagcgagatcatcaggcaaatgcaattcacaatgagatatcatggagggaaagtctgtttctcttgaactacttactttaaaaagtttaaaccaaaatatccaatgtagtggtctaatgaattctgaaatgaacaactatgctttctgcctattatcttacaatcaacatttttagctttttagcccaggtctaaaaatggctgttaccaagcatgtgtttttgttttttttgttttgttttggtttttaatggaatggtatcatgtactggcatgatctagaagtagctacatcagccctcttctggtaatgaatcatcagcacatataaatggaaggtaaagacaagattattttattaaaagaaacaattactaactcacagggcaacaaagcttcggcagctataggatactacttgtgagtatcctatactcctatactccaggtctctgccttaacccttcacacgtacaggactactgtctctcaccttgaccacattccctaaaagaacagagaactctgtagtatgaataccacagacctcagttactacaggctttgactgaaagaataaaaggtattaaatgaaagcacataatctgagccatgggcctccactgttcctttccttctccaaagtttcattctgccaaatgttggaagccaggccaaaccttggtttctggaaaacaattcaaaggcgctggccatgcctagtgtgtttatccttctttctgtttaaaaccggtcactggctcaattgcctcctgaacgaagttagcaactcccagccaggagctcaggccttgaggacgggctcatggctctgggacacacctctcaggactgccctccgtttgcccaatgctctagccaagcaacaacatggcagttcttagcacacctagcatttccttctctctttccttgcttcagctctgctaacacccttcctctgcttctgccacccatccaacacccggcttgagccagattcaaattttgttcatggagccatgcaatggattggaacatcaatatagttcaatacccaccaacagtaaacagatgacaggatccattctacactgcaggcaaagtcaacacacacaaatctggttaagatgtgtctttggatagcatacatggaaatatcaaaattatctaaatctacataattgattctaatagatctggcttctctaataaatttgtaaatgggaacatgcctctctcacccccaaatagcatatgtaatgtggatgtaattgttggcctcagctaatgatatatttttaacaacacaaggaatgatcatccatatttttatgaaatgtagatctgtaaaataaatacagttaaataatctacaagtaggtttacaacttaaagcctacagggacaaatatattttgatcttccaatagctaacactttgagcaaatggaggaaatactccaaattatgtaatactctatataatctctagagttagaatgagaatgtgtttaacatgtgctctgaagttaagcctatacattatgaaactttagacgttccagctttaaaaataaaaaataacagctttaaataacatttctaaatacaacatttggttactaggagtctctcatgattgaaatttacttagcctgaaagatgaaatgtcaaactccaaatggaaggaaacaaaattagtgcaagtctgtatctactcttccactagaaaaatggtttcactaagtgagtttactgatttccactcttggaggctagaagtaaagatagctaaacaataggaagaggtgcttccctaaagtaattaagaaaacaatgtttcactttactactatcctccaagcaccagatctatatatttgtataagcacagcactacccaaatatatataaaatgaaaatccactataacaaatttgtcaaataaaatctgagcttctccactgttgttcaggcagcaatactgcccacaagtatgagaaacttaatattgattagccattgtgggttaaaaattccacagaagtgccatattaaatcattcgggtagcttttgcttctggaaagcacattccagcactttgggaggctgaggcaggcagatcacctgaggtcaggagtttgagaccagcc

SEQ ID NO: 16786 - RNA, 66 nt, Homo sapiens
  source 1..66: mol_type = other RNA
taatgcattaaattattgaaggcctggggtgcccaagggccttcaataatttaatgcattaattaa

SEQ ID NO: 16787 - RNA, 2934 nt, Homo sapiens
  source 1..2934: mol_type = other RNA
taattgcttccatgtttaagaaaaaatctagtgtttattcgtttcttcaccacaatgaaagctagagtgaaattgttaggagagatggtttttaagtaggtcgacatctttttcgcttcatggtcaagcaatgcttgaagctgaccatctcccactccatcccgatacacaataacagaatgtggcatcgatgattcgtttttacaccagacatccagggcagctttcaagcagatctccagctctttcacaagctcttctcctgttttctggatgacacattgagagtaccactttgttaattcagcattggtacttgcaacaaatcctgctattgatttctgtcgatttacgatatcgtggaaacaatcaatgccaacgaacattgttctttgtacgtctgtctccaccttccagagggctcctcccatcttgcaattcatctgctgggcaatcttggtgacgatggtccttgcctggactttttctaaggtctttttcaccacacactggcttggaattgggcatttggtacataggtatctttttatgctgtcatatctacgtttgtcatcattgggcaggatacaaatcaccatctgcagtgttggtctagtatatttccgtaatgtgtctatataggagttagcatcaccatctacttcaatcatttctgctggtttcatagttatgcccatgggggctgtgacactctgtagatgaccctttaaggacatggcttctctgtgactgctcctgctatagagtatgagccaactatgtagtggcattgcattaagtaagggtaattctcttatttctcttgaccagtctccttgtgaattggctttaaccattcttctgccttgcacgatgtttgcgtttttcaaaactcttcccgggacggacaaaaaattggtatcaaatttcaaatcccagagttgaagtaactctcgtacttttttattatcttgtagagtattgatgaattcttttaatgtatgatgccttcttcttggactcaatcttgtatgtttagccaattctttcacaatgctataatctttacatatttcatctgttagacctgtcatgtggcacagctgaggaatcagcaggataggttcacgttgtgtacccgttaggccctttttccatctgccctggctgaccaaaagtggctgtttcttcactgtgacaatttctttatgttgctgcctgtagtagtctatataggtgattttgctgccatctgatttgttaaatgtgtcttcaggattctgcttccaatcaatatcatctactctgtaggttttgttgttgtattttgtcagaacaattgatccaattaatttattagttacttcctctcggatgtttcctgtctgggcctgggcagatgttctctttatgaaatcataagcagtttctattcggagcagtttgtggctcacatcggcacagagggtaatgctgttttcgtattgaagaacagaagtaacataaccaagccagatttccaaactggtaccatgacggtataactgaatggccttctttttggtataatagttgcgaccaacttgttcaaaatccagcagcttgaaagttcttctaaagagaatgttgtaatagcgtaggcaatctggcgacgtgggcgtgagttctttggaaaactcaactgtaatcttcacgatgtttttgtctttggttgtgctcaaccattccactctccgctcttttagtggccgagataataataaagagtttccatcaaatatatggcgctctccaaatttccttctatgttgatcaagtaaaattgtacggagatttccatcttctatgtctggtttgtagtcaacgttgtatttatatgcaacccactgaggacgagatatcactcggaagtggttggcgagtagctgtaccactgtaccctctgaacctgtttttgagtctttaacatgcttcatatcttgcctggtgttcaccaccaggtcttgaaaaactccaccaatccttctctcctgcaagggcgctgtatgcaacccagcctcaggtccaggttccttcaccccttgagactgtgctcctcctcctgctcctcctcttgctgctcttggctgcagaggtctaaccactgggacttcctcctgcagcggccggggtgtcgactgcaactgagggggctcctgggtctgaactagcttcgctcaacaaccaactctatgttcttttcagtacaggcacatatctcttgcagaaaggaaacaacgttacagggctcactgtagctgatccaggtgctctgggtcccccaggtgcctcttgttggtagctctccctgcggcgggctctgcctcgggcgcgagtccttgccctaccaggcattgtggtcctgaaggtgatgaccctgtaatcccagctacttgggaggctgaggcagaagaatcgcttgaatcctggagagagaggttgcagtgagtcgagattgtgccaccgcactctggcctgggcaacaacggcaaaactttatctggtcacatatttccttagaagcttcagtagtcagatcctgatacgaaccatgcacctcctccagccatgatgacgccggccacttccacagatggaaaaataattcaggacaagccactggagggggtcacaccacctgacacctcccagtccccctgcctcttttgccttccaaatcctccctttaaaaaccgctttggccgggcgcggtggctcacgcctgtaatcccagcactttggcaggctgaggcgggtagatcatgaggtcaggagatggagaccatcctggctaacacagtgaaaccctatctctactaaaaatacaaaaaattagccgggcgtggtggcgggcacctgtagtcccagctactcgggaggctgaggcagcaaaat

SEQ ID NO: 16788 - RNA, 2807 nt, Homo sapiens
  source 1..2807: mol_type = other RNA
taattgcttccatgtttaagaaaaaatctagtgtttattcgtttcttcaccacaatgaaagctagagtgaaattgttaggagagatggtttttaagtaggtcgacatctttttcgcttcatggtcaagcaatgcttgaagctgaccatctcccactccatcccgatacacaataacagaatgtggcatcgatgattcgtttttacaccagacatccagggcagctttcaagcagatctccagctctttcacaagctcttctcctgttttctggatgacacattgagagtaccactttgttaattcagcattggtacttgcaacaaatcctgctattgatttctgtcgatttacgatatcgtggaaacaatcaatgccaacgaacattgttctttgtacgtctgtctccaccttccagagggctcctcccatcttgcaattcatctgctgggcaatcttggtgacgatggtccttgcctggactttttctaaggtctttttcaccacacactggcttggaattgggcatttggtacataggtatctttttatgctgtcatatctacgtttgtcatcattgggcaggatacaaatcaccatctgcagtgttggtctagtatatttccgtaatgtgtctatataggagttagcatcaccatctacttcaatcatttctgctggtttcatagttatgcccatgggggctgtgacactctgtagatgaccctttaaggacatggcttctctgtgactgctcctgctatagagtatgagccaactatgtagtggcattgcattaagtaagggtaattctcttatttctcttgaccagtctccttgtgaattggctttaaccattcttctgccttgcacgatgtttgcgtttttcaaaactcttcccgggacggacaaaaaattggtatcaaatttcaaatcccagagttgaagtaactctcgtacttttttattatcttgtagagtattgatgaattcttttaatgtatgatgccttcttcttggactcaatcttgtatgtttagccaattctttcacaatgctataatctttacatatttcatctgttagacctgtcatgtggcacagctgaggaatcagcaggataggttcacgttgtgtacccgttaggccctttttccatctgccctggctgaccaaaagtggctgtttcttcactgtgacaatttctttatgttgctgcctgtagtagtctatataggtgattttgctgccatctgatttgttaaatgtgtcttcaggattctgcttccaatcaatatcatctactctgtaggttttgttgttgtattttgtcagaacaattgatccaattaatttattagttacttcctctcggatgtttcctgtctgggcctgggcagatgttctctttatgaaatcataagcagtttctattcggagcagtttgtggctcacatcggcacagagggtaatgctgttttcgtattgaagaacagaagtaacataaccaagccagatttccaaactggtaccatgacggtataactgaatggccttctttttggtataatagttgcgaccaacttgttcaaaatccagcagcttgaaagttcttctaaagagaatgttgtaatagcgtaggcaatctggcgacgtgggcgtgagttctttggaaaactcaactgtaatcttcacgatgtttttgtctttggttgtgctcaaccattccactctccgctcttttagtggccgagataataataaagagtttccatcaaatatatggcgctctccaaatttccttctatgttgatcaagtaaaattgtacggagatttccatcttctatgtctggtttgtagtcaacgttgtatttatatgcaacccactgaggacgagatatcactcggaagtggttggcgagtagctgtaccactgtaccctctgaacctgtttttgagtctttaacatgcttcatatcttgcctggtgttcaccaccaggtcttgaaaaactccaccaatccttctctcctgcaagggcgctgtatgcaacccagcctcaggtccaggttccttcaccccttgagactgtgctcctcctcctgctcctcctcttgctgctcttggctgcagaggtctaaccactgggacttcctcctgcagcggccggggtgtcgactgcaactgagggggctcctgggtctggaaggcatcgtgctacttccatgcagtatatggtccccctggaggttgtcagatggggccccgcagcgccactatggatctgtagctgatccaggtgctctgggtcccccaggtgcctcttgttggtagctctccctgcggcgggctctgcctcgggcgcgagtccttgccctaccaggcattgtggtcctgaaggtgatgaccttatctggtcacatatttccttagaagcttcagtagtcagatcctgatacgaaccatgcacctcctccagccatgatgacgccggccacttccacagatggaaaaataattcaggacaagccactggagggggtcacaccacctgacacctcccagtccccctgcctcttttgccttccaaatcctccctttaaaaaccgctttggccgggcgcggtggctcacgcctgtaatcccagcactttggcaggctgaggcgggtagatcatgaggtcaggagatggagaccatcctggctaacacagtgaaaccctatctctactaaaaatacaaaaaattagccgggcgtggtggcgggcacctgtagtcccagctactcgggaggctgaggcagcaaaat

SEQ ID NO: 16789 - RNA, 2724 nt, Homo sapiens
  source 1..2724: mol_type = other RNA
taattgcttccatgtttaagaaaaaatctagtgtttattcgtttcttcaccacaatgaaagctagagtgaaattgttaggagagatggtttttaagtaggtcgacatctttttcgcttcatggtcaagcaatgcttgaagctgaccatctcccactccatcccgatacacaataacagaatgtggcatcgatgattcgtttttacaccagacatccagggcagctttcaagcagatctccagctctttcacaagctcttctcctgttttctggatgacacattgagagtaccactttgttaattcagcattggtacttgcaacaaatcctgctattgatttctgtcgatttacgatatcgtggaaacaatcaatgccaacgaacattgttctttgtacgtctgtctccaccttccagagggctcctcccatcttgcaattcatctgctgggcaatcttggtgacgatggtccttgcctggactttttctaaggtctttttcaccacacactggcttggaattgggcatttggtacataggtatctttttatgctgtcatatctacgtttgtcatcattgggcaggatacaaatcaccatctgcagtgttggtctagtatatttccgtaatgtgtctatataggagttagcatcaccatctacttcaatcatttctgctggtttcatagttatgcccatgggggctgtgacactctgtagatgaccctttaaggacatggcttctctgtgactgctcctgctatagagtatgagccaactatgtagtggcattgcattaagtaagggtaattctcttatttctcttgaccagtctccttgtgaattggctttaaccattcttctgccttgcacgatgtttgcgtttttcaaaactcttcccgggacggacaaaaaattggtatcaaatttcaaatcccagagttgaagtaactctcgtacttttttattatcttgtagagtattgatgaattcttttaatgtatgatgccttcttcttggactcaatcttgtatgtttagccaattctttcacaatgctataatctttacatatttcatctgttagacctgtcatgtggcacagctgaggaatcagcaggataggttcacgttgtgtacccgttaggccctttttccatctgccctggctgaccaaaagtggctgtttcttcactgtgacaatttctttatgttgctgcctgtagtagtctatataggtgattttgctgccatctgatttgttaaatgtgtcttcaggattctgcttccaatcaatatcatctactctgtaggttttgttgttgtattttgtcagaacaattgatccaattaatttattagttacttcctctcggatgtttcctgtctgggcctgggcagatgttctctttatgaaatcataagcagtttctattcggagcagtttgtggctcacatcggcacagagggtaatgctgttttcgtattgaagaacagaagtaacataaccaagccagatttccaaactggtaccatgacggtataactgaatggccttctttttggtataatagttgcgaccaacttgttcaaaatccagcagcttgaaagttcttctaaagagaatgttgtaatagcgtaggcaatctggcgacgtgggcgtgagttctttggaaaactcaactgtaatcttcacgatgtttttgtctttggttgtgctcaaccattccactctccgctcttttagtggccgagataataataaagagtttccatcaaatatatggcgctctccaaatttccttctatgttgatcaagtaaaattgtacggagatttccatcttctatgtctggtttgtagtcaacgttgtatttatatgcaacccactgaggacgagatatcactcggaagtggttggcgagtagctgtaccactgtaccctctgaacctgtttttgagtctttaacatgcttcatatcttgcctggtgttcaccaccaggtcttgaaaaactccaccaatccttctctcctgcaagggcgctgtatgcaacccagcctcaggtccaggttccttcaccccttgagactgtgctcctcctcctgctcctcctcttgctgctcttggctgcagaggtctaaccactgggacttcctcctgcagcggccggggtgtcgactgcaactgagggggctcctgggttgtagctgatccaggtgctctgggtcccccaggtgcctcttgttggtagctctccctgcggcgggctctgcctcgggcgcgagtccttgccctaccaggcattgtggtcctgaaggtgatgaccttatctggtcacatatttccttagaagcttcagtagtcagatcctgatacgaaccatgcacctcctccagccatgatgacgccggccacttccacagatggaaaaataattcaggacaagccactggagggggtcacaccacctgacacctcccagtccccctgcctcttttgccttccaaatcctccctttaaaaaccgctttggccgggcgcggtggctcacgcctgtaatcccagcactttggcaggctgaggcgggtagatcatgaggtcaggagatggagaccatcctggctaacacagtgaaaccctatctctactaaaaatacaaaaaattagccgggcgtggtggcgggcacctgtagtcccagctactcgggaggctgaggcagcaaaat

SEQ ID NO: 16790 - RNA, 2751 nt, Homo sapiens
  source 1..2751: mol_type = other RNA
taattgcttccatgtttaagaaaaaatctagtgtttattcgtttcttcaccacaatgaaagctagagtgaaattgttaggagagatggtttttaagtaggtcgacatctttttcgcttcatggtcaagcaatgcttgaagctgaccatctcccactccatcccgatacacaataacagaatgtggcatcgatgattcgtttttacaccagacatccagggcagctttcaagcagatctccagctctttcacaagctcttctcctgttttctggatgacacattgagagtaccactttgttaattcagcattggtacttgcaacaaatcctgctattgatttctgtcgatttacgatatcgtggaaacaatcaatgccaacgaacattgttctttgtacgtctgtctccaccttccagagggctcctcccatcttgcaattcatctgctgggcaatcttggtgacgatggtccttgcctggactttttctaaggtctttttcaccacacactggcttggaattgggcatttggtacataggtatctttttatgctgtcatatctacgtttgtcatcattgggcaggatacaaatcaccttgaaaaccagcaaacatgacattcccatctgcagtgttggtctagtatatttccgtaatgtgtctatataggagttagcatcaccatctacttcaatcatttctgctggtttcatagttatgcccatgggggctgtgacactctgtagatgaccctttaaggacatggcttctctgtgactgctcctgctatagagtatgagccaactatgtagtggcattgcattaagtaagggtaattctcttatttctcttgaccagtctccttgtgaattggctttaaccattcttctgccttgcacgatgtttgcgtttttcaaaactcttcccgggacggacaaaaaattggtatcaaatttcaaatcccagagttgaagtaactctcgtacttttttattatcttgtagagtattgatgaattcttttaatgtatgatgccttcttcttggactcaatcttgtatgtttagccaattctttcacaatgctataatctttacatatttcatctgttagacctgtcatgtggcacagctgaggaatcagcaggataggttcacgttgtgtacccgttaggccctttttccatctgccctggctgaccaaaagtggctgtttcttcactgtgacaatttctttatgttgctgcctgtagtagtctatataggtgattttgctgccatctgatttgttaaatgtgtcttcaggattctgcttccaatcaatatcatctactctgtaggttttgttgttgtattttgtcagaacaattgatccaattaatttattagttacttcctctcggatgtttcctgtctgggcctgggcagatgttctctttatgaaatcataagcagtttctattcggagcagtttgtggctcacatcggcacagagggtaatgctgttttcgtattgaagaacagaagtaacataaccaagccagatttccaaactggtaccatgacggtataactgaatggccttctttttggtataatagttgcgaccaacttgttcaaaatccagcagcttgaaagttcttctaaagagaatgttgtaatagcgtaggcaatctggcgacgtgggcgtgagttctttggaaaactcaactgtaatcttcacgatgtttttgtctttggttgtgctcaaccattccactctccgctcttttagtggccgagataataataaagagtttccatcaaatatatggcgctctccaaatttccttctatgttgatcaagtaaaattgtacggagatttccatcttctatgtctggtttgtagtcaacgttgtatttatatgcaacccactgaggacgagatatcactcggaagtggttggcgagtagctgtaccactgtaccctctgaacctgtttttgagtctttaacatgcttcatatcttgcctggtgttcaccaccaggtcttgaaaaactccaccaatccttctctcctgcaagggcgctgtatgcaacccagcctcaggtccaggttccttcaccccttgagactgtgctcctcctcctgctcctcctcttgctgctcttggctgcagaggtctaaccactgggacttcctcctgcagcggccggggtgtcgactgcaactgagggggctcctgggttgtagctgatccaggtgctctgggtcccccaggtgcctcttgttggtagctctccctgcggcgggctctgcctcgggcgcgagtccttgccctaccaggcattgtggtcctgaaggtgatgaccttatctggtcacatatttccttagaagcttcagtagtcagatcctgatacgaaccatgcacctcctccagccatgatgacgccggccacttccacagatggaaaaataattcaggacaagccactggagggggtcacaccacctgacacctcccagtccccctgcctcttttgccttccaaatcctccctttaaaaaccgctttggccgggcgcggtggctcacgcctgtaatcccagcactttggcaggctgaggcgggtagatcatgaggtcaggagatggagaccatcctggctaacacagtgaaaccctatctctactaaaaatacaaaaaattagccgggcgtggtggcgggcacctgtagtcccagctactcgggaggctgaggcagcaaaat

SEQ ID NO: 16791 - RNA, 983 nt, Homo sapiens
  source 1..983: mol_type = other RNA
taattgcttccatgtttgaaaaagggagtctgttcttttgctaggccatgaggctggaatccacttggcatactgtgttgagaggtctaagttcagtggtgctctcagcagcagccgggaggtgtgattctgaggctgggtgacctgtgctttcagagaagcaggaaagggccctctaggtgtgctgcagtctctcagaaagagttcatcaaagtagcgagcaacgaaagaaactggtcttctttgatcggttttctgttattttcactggtccacctgctcctgctgaattgctgtcattcatttttctgttgagttttgtcattatatctcgtgcaagtgtaaaaaatgcctcttctacatttgcactggattttgcgcttgtctccaagaatttaatcccatagtcaattgctagcttctcccctctttcttttgacacttgtcttttgtcattcatatcacatttgttacccaggatcattctttcgacatcggaagaggcatgctcttcaatgtttctgatccaatttttaatattgtcaaaggatttttcatttgtgatgtcatagaccagcataatgcccatggctcctctgtagtacgctgtcgtgattgttcggaatctttcctgacccgctgtgtcccatatctgaagcttaattttctttccatctagttctatcgttctaattttaaaatcaattcccaacaccacagtgctataagtgacagtgattccaaatccaatactctgtccactacatcacactgcttcattagcagacattttgtgggataataaaatgggttgtttttattcctctatgtgaggccgcacgatggtggagatgaaggtggtgttgaaggcgtcctctgagaagcggaacaggaggcaggtcttgcctacccccgagtcgccgatcagcaggagcttgaagagataatcgtacgtcttcgccatcttctcgctccggccctct

SEQ ID NO: 16792 - RNA, 851 nt, Homo sapiens
  source 1..851: mol_type = other RNA
taattgcttccatgtttgaaaaagggagtctgttcttttgctaggccatgaggctggaatccacttggcatactgtgttgagaggtctaagttcagtggtgctctcagcagcagccgggaggtgtgattctgaggctgggtgacctgtgctttcagagaagcaggaaagggccctctaggtgtgctgcagtctctcagaaagagttcatcaaagtagcgagcaacgaaagaaactggtcttctttgatcggttttctgttattttcactggtccacctgctcctgctgaattgctgtcattcatttttctgttgagttttgtcattatatctcgtgcaagtgtaaaaaatgcctcttctacatttgcactggattttgcgcttgtctccaagaatttaatcccatagtcaattgctagcttctcccctctttcttttgacacttgtcttttgtcattcatatcacatttgttacccaggatcattctttcgacatcggaagaggcatgctcttcaatgtttctgatccaatttttaatattgtcaaaggatttttcatttgtgatgtcatagaccagcataatgcccatggctcctctgtagtacgctgtcgtgattgttcggaatctttcctgacccgctgtgtcccatatctgaagcttaattttctttccatctagttctatcgttctaattttaaaatcaattccgatggtggagatgaaggtggtgttgaaggcgtcctctgagaagcggaacaggaggcaggtcttgcctacccccgagtcgccgatcagcaggagcttgaagagataatcgtacgtcttcgccatcttctcgctccggccctct

SEQ ID NO: 16793 - RNA, 1940 nt, Homo sapiens
  source 1..1940: mol_type = other RNA
tacacaagaaaaccaaggctcagaaaggctttctgaaaatccaacactgcatgttctcattcataagggggagctaaataatgtatacaggggagctaaataagggagagctaaataatgtggatgtagagtgtggaacaatcacactagagactaagaagggttggaggttggaaggggttgagggatgagaaattacttaatgggtacaatgtacattatgcaagtgatggtcactctaaaagcccagacttcccctaaagcaatagatccatgaagccaaactgcactttaccccttaattttatgcaagtgtttaaaaattaaaatgaaaaaaatacaaacacgggcttgtgtgattccatagcacatagctttatcccaaggtaagggggcacaccttaagacagcccccactttggtgaaggctgctagtttctgggaagctagcaaaacatttctccaaccaaattgcggaaaagctatatataccacgtacactaataataaaaaattgccaacatgaatctccaagctttagttttttaaattgtcagatgggtgcataggtgaaggagacaagaaacactggccaggggagactctcaagatactggaaccctcgtctcagttctgtcttaataaaatttttgcttttgagttaattgtttcatgcctatatgctgtctatggtaccctcttagtataagaagtctagacataaaaaacctctacaattcaattaatatgtgtgtgtgtgtgtgtgtgtgtgtgtgtgtgtgtgtgttcacagattatagagattcacagctgacaaaaaataacttctgggagataattttctagtgggaaagaaacatcaacaattcattacaaaccaataaggtcactgtcaagataagtgtgtggggacctccaaggaagctctctattttactaaagtccagagagtctgtcccgggaaggcttccagactgcagctcattggtttattcagccagtgtgtactgaatgctttttataagctttgtcctcattgaggttctggaaataaatattgtcaataaagcatggcccctgccttccatgaggcaactcacaatctctgctaaaccccagggaaagggtggttcagctactttttaggaagaattctggaagaactgagaatgtttacctcttctaacagtcttctctcattcacgtttaatttaattagaaatggtctaaattgaacttcggcagagcaaagcaacaaaacaacctgagaaactctatttgttaatagggtagatttaagtcgatgttctctaacacagtaaacataagcttaaatgttccctaattagagatagtgtgaacccagcagagaataccaagtcctatggggtgagcccacagagtcacatgtgctcagagtcacatcagtaactcagcatcatacatgacacattcaaactcactctgcatgcaactggtctgtagatttatttttatttactgattttctgcattttctattcatatttttaagtagaattctaacagttttactgtagacttttgccttacctcagttggtacacaattccaaaattcacctatctcactaaaacagtgaagaaccatgatttccttactgttacaattccccacaaaaaacaaaaatgaatcaggtcattgttacttaagtgataagtaccttagagaaagctttttaacatacaatcacagatcccttgttgaagaacacttttgctaacagttttgccttgctgaattaggaaaaaacattctttcaaggacagtagtaagattgaccaggtttctttgtactctctatatttgaagaaattgagccagttcagtccaagtcacttaaatcctgagtcttgattgcctaatttgtaaaactgttcagcttcctgccagactcatag

SEQ ID NO: 16794 - RNA, 87 nt, Homo sapiens
  source 1..87: mol_type = other RNA
tacacaagaaaaccaaggctcagaagctccctgacagcccagggtcactgagtccagaagcagcagaggccgaccccaggctgagac

SEQ ID NO: 16795 - RNA, 789 nt, Homo sapiens
  source 1..789: mol_type = other RNA
tacacaagaaaaccaaggctcagttgttgaagtgtcttgctcaaggatgagcagctggggaaggggaggagtccgcctcacccttcccattgcagctggattttggaagccaattccagctggaggactaggagatttgtagtgggtgagaggagcaaatggaggattttaatacaagagtgaagtaatcacagggcttctctagaaatgttggtccagatcaggttgtaccaaggatttaccaagaatgcatgaatagtgacgtggctggtgtggggggtgcaggatgtctggggagacccgtggaaggtgctggaaggaccacttgggaggactggaggcaggtgaaacttgctcatgaaaactccagccatgcagctgggccttggggctgggtggaggggcattgggagcatctgcctagaaggagtgggtggtgaggactgacattcccaccctcccctacctgggtggcagggataagtggtactgaaagggccccttacgacatgtgccccaaagcactgtgacctcagagtttccaggtggtggtcaggtcccctgggtccaccaagggcccctctgggtcatcttgccgctgtccttgaccccatggggctgcccctaggggctaccttctctgctttaaacctcacttcccttccctggccccttatataaaaacaaagcagaaccaaccctttgcaaacacacccgagagctggaggaacaggtcttggggcatttgctgttgccggatttactgtgtgctgcttttgtcttggaaga

SEQ ID NO: 16796 - RNA, 3837 nt, Homo sapiens
  source 1..3837: mol_type = other RNA
tacagatgcagattctctgacttctaccgtgtatcctgaagaaaagacaaatgaaaacactatggcttttgttatttacttccaagaagaacatttttctgtttattcttagaatgtgaattttttttttcaactcagggccaagtacaaacttttgatttttgaaattttttcaactcagggccaagtacaatcttttgatttaaaaattttttttcatgaacaaaccatcagtagttattaaggagcccaagaaataggagatgtgaaagcaggatttctttgtgtttcctttgaatgttgttattttgagtattatcattatcaggtagaggaagaaaggtaggctgggaagtaggtccttatgatatcttgactatggatcccagatttacatttcacctgaattgtgacaccacttttcttggctgagaactttggccttggtgccacaaaataagatgatgaggctgattcttgctttggcgaggtgggaatgcccacaggcactggggatgcactgactggtgaggaggcctctgcaaagaaggaaggaggagaggtataggctggtaccgagtacactgacgaagcctgcacattcgtaggtgaggcagcattcactggccggggaggaagagcttgcttcatggccagggctgaattgaccttgactgatgacttctgggggaggccatcctttgcatctggaggttggaaagtaaacaaggatgcattgagctgatacggttggtgcttcatgacatctaatgcattgaggggtttctttccctttttcttgcccattttggagggctgtgcagctgatggctgagacttgagagcagccagtgggtaagacggcgagtggataggattataggccacaggaggaggtgctcggacattggaggagtacttccaactggccgggagagatggagtgggagactgagctcgagcagcgtgggcctgcaccgtgtctgaatcgaccacatacttctccattctcgactgccttttagcaaagagctgagctcctctcccactcattcctggaagctcattggatggtcccactgcaccaggctgaacagcattgactgttggtgtggaaactgttggtttgggtgtgtaattctgactggctactgctgcttgtggtcctttgaagggaccagccacgttcaaagtacttgcaggccgggcaggagggtaagaaggctgggctattttgatggaggagacaacggtgccctttgatgggttggatgtggggaaggcaggaggttgggtgggagccactcctggagaccagactggggaaactggagttactggttgggaggatgaggacttgactgcaggttttggagcaacaggaggaggggtcttttgtttggcagaggagctttgcatgaaattacaagcctctgcccccaagctgaggtagtcttcttccggtccggaatcacctccagctccagtgccccgtttgccttctgaattttgaaggagtgacaagagttcaggatttgggcttactttgggctctttaaaagtaaacatgggttttgtcgtgcttctccttttggcctcctgcaatattcctgttctttttgctggcactgagatcctctcatctcgggaagctattcgctcagacgaatcgtaaaaggctggctgggaccacggggcaggctggggccatggagggggctgtgctgggccagcaatcggacttgaaacccctctggagaaggcgtcagggggaggagtgactgcagagtaaggtggaggtgcaggaaagtcagcaatgggactcgtcatgtttcgggttggcgagaagggggtagctggctgattcacagaccctgggaagggtttggccgttctattcatggggaccatcctctggatgtttgctgtctcagatgtcccactgaagccattctgttggggaacatggccaagaccatgactcacctcgatgtagcttttgctcacagagctctgcgttcttaccgactcttcctcctttctttggtaagaagtcgtggttctcaggccatcggtctgggcagcatcttgttctctgcttggcgttccacctaccttgtcctcttctttttgggctgtgatctgatccattctctccctcctcttggcaaacatgagggctcccttgcctgtggtgtctggtaacatctccatcttgtcccctctgttcagtttcttttcaatgtccaccagtccagaatcccagtcaaagttcacaacttgtgtgttgtcgtcaacgtcagacaataactcttcatccacctctgattcgcttgcaccaagaaatgctacttcacatgtatcctccttgtcaccttcttcctcctcgtccgcctctcgctcaagctcgccagtaccgtagctaactagggtgtatttcctggccctccgacgtcgcttcttaaacatcaacacccccttggagttggggttgggagcatccgttagaagaagggcaatgcttttgcatttagattttgcttccttcacttgtttttctgacaggctttcactcctcctgagccgtgcatgccgcgctcggtgcttgtgaggtctgctgtgatctttttccgagcgtggatcttctccctgctctgtgccttctgatgagacggcaaaggataccagagaaggaggtgcttctgactgccctccttccactggagaatccacacactcctttcctgcctgaagcctgcacccttctgtcttctgcctgtcagagcagtcgaggatcacttccacccggggcagtcccgcatctcctgcttcactttcctggatcactctcaactctctgccactggagatctggattatcttgctggacctcaggaaagggtctgctttctcattagtagggatcgaatttatgtggacaatcctgtcatgtgacaagttagggtctgggtcaggagacttagatttttcagctcccgggagagccactaaagggccactagcgcccttatgtctctcctgtgaaagggacagttgcagctcaaccacaggcccaggctgtaccgcttctaccttctcccttaagatcagctcttctgccacgcgtcctctttgggagtcaggcatttggggagccctttggtagctcgggcctgtttcttctttcaagctgcctgcacagtcgggaccacttctttggttctcagctaggggaacttcagtcttgacaggggcgaggaagaattctgtgcactgggtctttgtggccggtcgaatctgcagggtggtactttccacataacccccatgtgtgagatgctcgaggtttttgttttcattttcagatatcaaagcctcacttattccactggatggtcttttgatgagcatttggagagagtctgttatgctttccatgagcttgatgacttcagggtaggtgagatctgcacaagggttgccattgatggaaaccacttcatctccctcacagagcccagacccagaggctttgctctgatttcgaatctttgcaacttgtaagggctgcttctgctccttgccaccttgcaatctgaacccccagggcgcccctccagtcatggaaatgcagataaaatcccctgtgcccatgttttccttttagttgggcagcatgaagagcttgacgagacagacgaagcttgggtgcggtagaggatgcgcactcagcttcgggcgcctgccgaggacgcaagactgggtaatgcagagcgtccgccgctgctgcagccgctgccccagccgccgccccagccgcctgctgcgaatttgtgc

SEQ ID NO: 16797 - RNA, 8921 nt, Homo sapiens
  source 1..8921: mol_type = other RNA
tacagatgcagattctctgacttctaccgtgtatcctgaagaaaagacaaatgaaaacactatggcttttgttatttacttccaagaagaacatttttctgtttattcttagaatgtgaattttttttttcaactcagggccaagtacaaacttttgatttttgaaattttttcaactcagggccaagtacaatcttttgatttaaaaattttttttcatgaacaaaccatcagtagttattaaggagcccaagaaataggagatgtgaaagcaggatttctttgtgtttcctttgaatgttgttattttgagtattatcattatcaggtagaggaagaaaggtaggctgggaagtaggtccttatgatatcttgactatggatcccagatttacatttcacctgtcacagagcacacataatttagataaacatgtcaagaatgacataaacagaggtaaacacaaggagctttacatttggaaccaaaaaataaaaattagaaaaattattacctatattaataacaaaaaaattacttaaactctaggaccctgtaggagtctagctttctcccctgtatacttgggatgcactttattggctggcaaacctttgataaaatcagaagtttgagaaatgtttgacaggacttgatatttaaaattaaatttctctttattcaattgcctctgagtagtgctgtgatttccaagtgccaggtagttaggtgtacaaatatacataccacagaaacatacagtttttaaaaaaattaagaaactggctgcatctgacgacatcaagaaaaaagataattctgattcaagggcttctccagaagatggggtttcattggcatgacgctcataggatgacctgtcatttttgtactattttttctagaaccatagagggatgacagtaactggcttcttagagcaattttgcctggtgtctggatcctgtgggaatttattagcctgctttgtggcccttggccaaccctggtaggacatctagagaagaattcaattctgctttttcccagaataattgttgactaactcggcaacaccaaagtgtcacaggcatctttgtgtcccccagagtccaatgatatgtggacccaagaccagcgagggtcatgtttctgggaatacagtgttggttcttagaatttatatattttttctcatgaacttataaaaatgtttaaaaacaaactcaacaaccctgattttaaagagaatgagcacacgccccacgacttccctctagaagcattttaagcatttagcttttcaaaaaacaatcatttctttttgatgaccatgacttcaaatgccctgcctgctgggccagttgtgactcatcaaatagcaactgatttcaataattcacccttagaatgggggtgcttgcaggagccctagtttataactggatgaaatgatacgcagccaagggcctttatttgagaaattaaatctaaacgcagacactaacagccatgtgtcttctgctcttaggagggtttactgtgaaagagccacacagagtgttcgacatgcctcttagcagccgaatgaccttcaaagttctttaaccttgtaactgcaaataggaaaatggtctcacatacgttagtctaccccctttcaatgtagatcaggtgttttttttttttttttggacatctcagatgtgactcttgctgccaggctagaatttaggctatgtgataattctcagctgtcctacaatgcctgcttcttgaaagaagtcggcactttctagaatagctaaataacctgggcttattttaaagaactatttgtagctcagattggttttcctatggctaaaataagtgcttcttgtgaaaattaaataaaacagttaattcaaagccttgatatatgttaccactaacaatcatactaaatatattttgaagtacaaagtttgacatgctctagagtgacaacccaaatgtgtcttacaaaacacgttcctaacaaggtatgctttacactaccaatgcagaaactgtgtttgttttcctctctaaaaaacaggatgtgtcaaaatgataaatattctaagattaaagtggcaatgctcagattcccaatcttaccagttctgggattcactctgccctcctagaagactgaggggaatatgctgtacttacatgtccatggaaccttccttcctcctagaatcccaagcgttatgcagattcattatagcacaacattcccgtcaggaagagaggtttgacacatgattaaggggaaacttgtggaaagagaaatgtttaaggtcctgcagaaagtcagtgactgtaatgacctttttcatttatattccagtgcctgtatttaaaccatgcagtggatttgggataatatacataaggcacctaacataacataggaactcgtaaatgattgtcgctcttgagctggcaatgaaaaccgacttcgtggatgctctgcctagaaattatgctaaggacaaaggaagaggcaaagtcctaaaaactaaacaaaaactgcctccctacacctcataaccagcggaccaaccaatcaagctaataccaacacagctaaggcaacaacactcagattgaaaatgtaccccatgggagggaggctgacgtctggaggtctaactctcccttctgtcacactgacatcacttccttggccccaacctgaaaggtggcacatatagcccctggtgggcagacagggaaagcaaattcctcttactccagggagctggttagtccttcttcctcccacttcccatctccctcagagtgaggtcagactttgttgtggatattgttttggagaacttccaccctcttctataaagtgggactgtatggtccaagatgagacctatgctgccagtgcccagctgaagttgtagatgcttttactgcatgcctgacatgcctcttacaaggttttggagaactccaaatagtcctaggatgaccagaaggcatagtcatgttatttgcatctttagttatcaactccaaatagtggctctgctaagattgccacctgtccaacaggaaatggaaagaaaacacttctcattcctgcataccacaccactagacaactggaaatacttctgggtcattaccatcctaggatacttttaagccgatgatctcaaaccgactacctgtgtgttccatgtctttcctctaattcatgccgctctttaaatgctatgttaagaatgcaaagctataaaaatgatcttttttcctgctgcaccataagaagccttttttggttgttctattagaaaagaattcaaaatgcaagcattcaacagatttcctttgcagggaacaagtaatacaaacaactgtgttatataatgaatagattgcttttttcctttatcctgtattaatcttaattggtttcccaaaaaggcaaataagagaccaagctacatcctgtggttgtaacctctaggtaaatttccaccaaaagcaatgaaagattttccagagaaaaagcagaagaatcagccccattgttctgcagctgacttaattctcctctttatgttttagaaatacctaaggattacagttttacaatgtatggagaaatagatatgctaacaacaatgaaattgttgtgggagccatatagagaaatatcagagaaattatttagatcagaatagctcatacaaggaagatttttttaaaatatggacattgaacagataaaggagacagtaatattttaataggatagtgaaaaatatagcagattgacagtgacagcagaaaaagagcaggaatacagatattttcagaagattaaaatggtactgtgtaccctcaaaccaggcaagtttttctgagaggtctctaaacatatctcctgcatagagtagatgatttttcttggagctgtcataaatgctttatagttctctacattaattcatgtcgaatattttccatggttggtcagactcagacttaaaatagatctgagaaaggtcttcaggtttactttcagtaccattattcacttcatagccagctgggtgacaacatggtgtgtggccaattaaagtttacaaggtaaccttgcctgaattatcctggtccatcgaatacaaatagtaaagtgaaggtgagagaatagaattgcaaggaacgtgggagaagcagttgtcaaaaagcaaagcaaacacaagaaaaaaaatctgtgagatcactcagaaatgatgctaataattgtgtgctctcaccctacagtctccacacacatggggttcctcgtgcttcacaatcagcccctgtagtcagtcagtaaaccttcaggtcccaatcatgtggtttctccaggtgaaacaatagccatgtacacctttatgtgcgtcctgccttttacatgttacttcgttatcctgtatactctaccacttgcctcagctgaggaaaacaaacttatgctttcatgggcaactggagatgtactcacttagttccttaagtaactggggagggagggtgggaatcaacctttaaagataattatccttctttccttatcccatttacttcattattactattattattattattattgagacagggtctcactatgttgctcaggctggtctccaactcccggcctcaagcagtcctcctacctcagcctcccaaagtgctaggattccaggcatgaaccaccatacccggccccatttactttaaataagttttctgaaatgagtttatatatgtaaaaacatctggcaaagaacctaatacataataagtgctcagtaattaagaccctctttcttacccacttcttactaaactatatacattccaacaatcctccgagtatcttctctgtgatatcaaacaggtggctgagattgacagaccagagctgctccctgtccttcatagattccttattcctttaacactagtaatagagataaggcactacctaaaagggaaatctcagtcaatataggttataccttcactacatttgaacctttcaccataggaggacagctgttatgttacataaaggctgattcctgatgtttgatatcactgatcactgtctttcttgtggctacagcacaaatcctaagtctcctgcttacttaatataacggtacatgtctattttggggtgctcctggattttttaagtgtgcaaagaagataaatatattttaggtcaatctgagttggatttttgactcattaaaaatattatactccttggacccagattaggaggtgacatatctgaaattaagtaagttgaggactttgctaggcattctcagggactcaagaaacactgcaaacaattcatttcaagcaaagtggacactcagcttcagctacaagattactcttccacaacagatggtttccacacctgaattgtgacaccacttttcttggctgagaactttggccttggtgccacaaaataagatgatgaggctgattcttgctttggcgaggtgggaatgcccacaggcactggggatgcactgactggtgaggaggcctctgcaaagaaggaaggaggagaggtataggctggtaccgagtacactgacgaagcctgcacattcgtaggtgaggcagcattcactggccggggaggaagagcttgcttcatggccagggctgaattgaccttgactgatgacttctgggggaggccatcctttgcatctggaggttggaaagtaaacaaggatgcattgagctgatacggttggtgcttcatgacatctaatgcattgaggggtttctttccctttttcttgcccattttggagggctgtgcagctgatggctgagacttgagagcagccagtgggtaagacggcgagtggataggattataggccacaggaggaggtgctcggacattggaggagtacttccaactggccgggagagatggagtgggagactgagctcgagcagcgtgggcctgcaccgtgtctgaatcgaccacatacttctccattctcgactgccttttagcaaagagctgagctcctctcccactcattcctggaagctcattggatggtcccactgcaccaggctgaacagcattgactgttggtgtggaaactgttggtttgggtgtgtaattctgactggctactgctgcttgtggtcctttgaagggaccagccacgttcaaagtacttgcaggccgggcaggagggtaagaaggctgggctattttgatggaggagacaacggtgccctttgatgggttggatgtggggaaggcaggaggttgggtgggagccactcctggagaccagactggggaaactggagttactggttgggaggatgaggacttgactgcaggttttggagcaacaggaggaggggtcttttgtttggcagaggagctttgcatgaaattacaagcctctgcccccaagctgaggtagtcttcttccggtccggaatcacctccagctccagtgccccgtttgccttctgaattttgaaggagtgacaagagttcaggatttgggcttactttgggctctttaaaagtaaacatgggttttgtcgtgcttctccttttggcctcctgcaatattcctgttctttttgctggcactgagatcctctcatctcgggaagctattcgctcagacgaatcgtaaaaggctggctgggaccacggggcaggctggggccatggagggggctgtgctgggccagcaatcggacttgaaacccctctggagaaggcgtcagggggaggagtgactgcagagtaaggtggaggtgcaggaaagtcagcaatgggactcgtcatgtttcgggttggcgagaagggggtagctggctgattcacagaccctgggaagggtttggccgttctattcatggggaccatcctctggatgtttgctgtctcagatgtcccactgaagccattctgttggggaacatggccaagaccatgactcacctcgatgtagcttttgctcacagagctctgcgttcttaccgactcttcctcctttctttggtaagaagtcgtggttctcaggccatcggtctgggcagcatcttgttctctgcttggcgttccacctaccttgtcctcttctttttgggctgtgatctgatccattctctccctcctcttggcaaacatgagggctcccttgcctgtggtgtctggtaacatctccatcttgtcccctctgttcagtttcttttcaatgtccaccagtccagaatcccagtcaaagttcacaacttgtgtgttgtcgtcaacgtcagacaataactcttcatccacctctgattcgcttgcaccaagaaatgctacttcacatgtatcctccttgtcaccttcttcctcctcgtccgcctctcgctcaagctcgccagtaccgtagctaactagggtgtatttcctggccctccgacgtcgcttcttaaacatcaacacccccttggagttggggttgggagcatccgttagaagaagggcaatgcttttgcatttagattttgcttccttcacttgtttttctgacaggctttcactcctcctgagccgtgcatgccgcgctcggtgcttgtgaggtctgctgtgatctttttccgagcgtggatcttctccctgctctgtgccttctgatgagacggcaaaggataccagagaaggaggtgcttctgactgccctccttccactggagaatccacacactcctttcctgcctgaagcctgcacccttctgtcttctgcctgtcagagcagtcgaggatcacttccacccggggcagtcccgcatctcctgcttcactttcctggatcactctcaactctctgccactggagatctggattatcttgctggacctcaggaaagggtctgctttctcattagtagggatcgaatttatgtggacaatcctgtcatgtgacaagttagggtctgggtcaggagacttagatttttcagctcccgggagagccactaaagggccactagcgcccttatgtctctcctgtgaaagggacagttgcagctcaaccacaggcccaggctgtaccgcttctaccttctcccttaagatcagctcttctgccacgcgtcctctttgggagtcaggcatttggggagccctttggtagctcgggcctgtttcttctttcaagctgcctgcacagtcgggaccacttctttggttctcagctaggggaacttcagtcttgacaggggcgaggaagaattctgtgcactgggtctttgtggccggtcgaatctgcagggtggtactttccacataacccccatgtgtgagatgctcgaggtttttgttttcattttcagatatcaaagcctcacttattccactggatggtcttttgatgagcatttggagagagtctgttatgctttccatgagcttgatgacttcagggtaggtgagatctgcacaagggttgccattgatggaaaccacttcatctccctcacagagcccagacccagaggctttgctctgatttcgaatctttgcaacttgtaagggctgcttctgctccttgccaccttgcaatctgaacccccagggcgcccctccagtcatggaaatgcagataaaatcccctgtgcccatgttttccttttagttgggcagcatgaagagcttgacgagacagacgaagcttgggtgcggtagaggatgcgcactcagcttcgggcgcctgccgaggacgcaagactgggtaatgcagagcgtccgccgctgctgcagccgctgccccagccgccgccccagccgcctgctgcgaatttgtgc

SEQ ID NO: 16798 - RNA, 93 nt, Homo sapiens
  source 1..93: mol_type = other RNA
tacagatgcagattctctgacttcttactgcaccagtgaagtcaggatctgcatttgaataagaccccagacaatgcctattgaagtgtgaga

SEQ ID NO: 16799 - RNA, 1460 nt, Homo sapiens
  source 1..1460: mol_type = other RNA
tacagccctgtgatctttccagcacaatccttttaaaacctctgagtcaaccgctctttgacctcagttgagcctccaattgattaatcctacttcctttttgctatctcactttcttcgttggttagctcagatttcaaaggccaacatggtaatcaatgttgtgtttataccctcaaatttctcactctctcacctatttggtgcttgcttcagtgataaaggggggcaggagagggggagtcaaaggcccaggcatgggacagggcagccatctagggtccaagacctcactttcaattcatgaaagggaatctttcttccccatgcctgctgttttcttccatgtggggacatgaactagtgtcacactcctggcttccttctactctcccacttgcccttctctactgcactcctgccagatggaataacatacctgattagtggctttggaaggagaactgagcctgcaccagatggggacaccttccttgcctctctcctcttggcaacaagcgcctacaaggagccactcatttcctgacctatttcctccatgctgttagtttcagagaagcctctcttggagaggtctgggagggttcactgaagcttgggtctggatgggtaagcctgtctaattctggtattcagtaagtgaaaggtcaaatctaagccacatttcccagctattaatgtctttccttctaaagggagcttgctgccttcgatgagcattgatttccctctgttcatggaggatgaaggcaaaactcccaatggaatcaaccttttcttctctccctctctctctctttctctcttgtctctacccaccaaccagtctgtccctggagagaacgtgccctcgactgcacctctgcaccagaggcttggataggtgcaacacaaatgcttgtcagatcaaataaaataatgatgttattatgtcttaaagaagaccatgtttgaggggtaagagaaaaatggggtctggagtttggtgcttaatcttaaagacccaacaataacatcaaattttaagtgatctcaaacccttcgtgctgcctggcaattccagctgatttcctcagtcaactcactcttccagtcaagagattatttcactgattcttctctcttctcaagccctcttgcttttaactcttgggtttgcttcttattttccactcacgacacggaaattccaactgtaaagactcaagtcttttctggagggggatcacacatttggctcttaaggattgtgctaagagttaagtgagatgttctgtgttcaagcacctagaaaaaataagaactccaatattagctattgctgtgagtgaattgtagtcagtccacagatgataacactcgccttcctcatttccttggggtcatctcttttgactttctgctgccttttcaaaacttttacactgtctaaggacaac

SEQ ID NO: 16800 - RNA, 3520 nt, Homo sapiens
  source 1..3520: mol_type = other RNA
tacagccctgtgatctttccagtttaactctgaggggcaccttattgtaaccctttctcaccccagtactggtaagttagtatagcaccttgatattatgttgacatatgggaaaaacttaaaaccctcattaattaaagtcctgtttatatttttgttttcagctcaaatgtatgtgaatgtatttaagtgccatgtttccaatacacatctatctttttgtagtaaacgataacctcacttggcattctcagaaaatggcacttctaattgaggcctggggtattacttaaacttacaatggctatctttcaaatccactataattaaaattcatgactttcctgcagctaatgtatactttgattccatcaaggttttctcatttccatcctggcctaataaaaaatgtcatctgctaaattactggcatgccttactgcatctggatcttccttagtttcaatacaaactttgtccaagcacttaatttcaggatggagaattcatgggaaacatgccactactccttactctgttctccaagacagacatcactaactaattatagtagtccggcctccggctagatgtgggctgaatccagatgtgggcttcttaaccttttgtttccaggtgagtagaattgcttccagtattagagttggtgtgccagataacgttagctttgggttccttgtctgtcttgtggcatctgacaagatttgtcatttattttgagtctagggatttttttctgaaagtaattgtctactgaaagttttctgaatcaggaaagaacaagttttgtgcggctcccccaacctgccacctttattcttatgaatctcctcctcaagacataaaattgccaaatatcattcataaaggcctgaaaaatagcgaggtttgttaaggaatttgctcagttagtccaattagtgtccaagattaacataaactttactgtaaggtttttaaaaacaaagacaatagtttggtttttaaattaataaaaaatgtaatatttcttatcacaaaatggatgaaattcttagtataaatccattgtacatgaatgatttaactttgaatttcttccacactaaatgaaactcatttggtttagaaattcggagataaaatcctactgtgaacttttaagaagttcatgattatttgttaatacttctgttgctctatgatgaaagtaaatgtgaaacatcagaattttacagatgatagattaaagtgcttaaaattattggtgaaaatgttagcattttaagagtgttttaactgcttcttcagttcataaccaggcattggtttaactctttttgactgtatattactgtactggctgaattgagaaaaaagagaagaaagctgtataaggagactcaaaatacttccatttgtgaaaataggtaagttagaagagttattatatttctgatgttcaaaccagacttatttgtatttttgggatctgaaggttgataaactttcaaaagtccaaatatcacattcctccaaactatccccatttttgaatacacgagcaggttttgtccaaagatgagttactctttcttctatctcattttagggttgaggacgacagtgaagaaaagttctcctccttggatactcttatccagctctttaggaccccctggatattctttgtagaaaatggtgtgagtgaaaagcccacaggtttgtcttgggagaaccatgatgtttttgtggataaaacccctccggtatctagctggcttcagatgtggatattcttcagtgctggtgattttaatattccagaccttcttccaggcctcataaagctgaacatgtacagggtagacgcccgaatggtgaggggccacagcgtagcccatgtccgttggaatgccgtgctctaaggcaaattttttgttgagaatcatctgctccaccaaagatgactcattgtggaagaggtggggctgcatatggctccacatgtgaggaaaccaccagaactcatccacagaccccaacagacagtcatctccttcatcttcctcttcagttcctgtatggtaaaatttccctgaaaatcccaggttgaatgtaaaatttgtgatttgtgcacgcaaaagattctgagtatcaagcagggcctttacatcattggtgttcattcttgttccctcttttcccacaaatatatcatcaatatccacaagaatgtacctgtccaaggacaatgtcagcctcttccctgataagaaggagatggcatctatgaagatgagcttgtgcagccaaaagttcaagttgttgccaaaaagaaccctttgaattccatcatgaagccccaggtcatgtataatagtggcataaaaagcacctttagagatggaaggagaaaggttttctggggtctttactttggcaaatattactggttgataggctgaatgattaatctgaaaaactgtccagtcagttccaggtaaagaacctttttcaagcttggaagatttggtcacacgaatcaatggagaatgaggattaatacaacaatcttttactgcaagatttccatatatggaaaaagggaaaccttttaactgaaagctctgtacactcttctcactagttttgtggaatccaatgacacccacaccatattctacacagtatttatctagaaggcttcgattccaggaatccatatttatatactttaaaatattctcataaataatgagaatgtatttgcctttcattttgtctataagcactgggagatctccctttccaggggcaatttcaatgtgatactggaatctacttgattctagaatcataatgatgtcttgaccaagagatgagtactggctctctacaaatactaggactgtggggtctgtccttgaggcatcaaaaagcttcattgctttcacttccattagttgatatggtaggtgttggaggtcgccacagtcaacttctgaagccgtctcagagagttcattttcctgtttgtagccactgtacaggtagtaagcagaaatgataatgctcaccatacaaaaagtggcaagcagaatgactgttctttgaaagtgtctgtgaagcttcatgataaaactcatgttgtaggtgctttccccaactatgccaacagaagcaccataaaaagttaaaagaaaagatggtgttccagctacttttccaatctctgtcaagagtttatgtcaccattgcagctcatttgtatcacttgatcaggactcacagaaaatacagtctggaattaaagttcagagctgaaaatgcttgagaaagttgcaatagatggaaaagaaacggaaacagtaccactcgttaccatcggctcaggctttttgactttacaagtggtagcaacaccagtcctggcccagtactctcatgttatgtaacatcttattaatattagccatcaaactgctaccaagctggtgaggcactagagggcaagagt

SEQ ID NO: 16801 - RNA, 3280 nt, Homo sapiens
  source 1..3280: mol_type = other RNA
taccattagaagagctggaagacacagagagtatgaagagagttgggaggaagacatggtgaggctcagcgtggatgcattgcttcctctgatttgcgtggaggtcacagacacactgctgagttttaagctcagagtgttaccattcaatatctcatctgaagaactgattagcagactaatcactacttacaactcttcaattccttctatccaatgttgaaaaaaattccatttgaatgggataattagagtagcccccacttaggacgtaaattgtaccccactgcagccaggaccagaatgctatcactctcaggaatgaaatcattcagagcatagctgcatcgggggcatgaccagcactatcctctccctgaccgtattccctgacctggctgcacaacccacttgatcgaggttaatgcaagccatctttctcctgaagacagtcactccctttgggcacatttaaattaaagcacctatcagaatgcaagtccagaggccctggcccatccgtcacagtgtatagaacggtctctttctacagagtaagagtgaccctatcctggtgcctttaaatctaaaaactattcagttcctttggtgggcaatcttcctggaagcactgacaacttcctctcatgggtgaaccattggcttaagctttcaagcagggatccaactggatctccctgaaaccactgccacctagctgcaaagcatgcaaccgggtgctctaggaagcctggtgttgcaaagaagggaagggcaactctgtcaatgtgcccaagggccacctgaaatgaaagtcatgagcagcctgggattaagcacttttgttgtagtcttcataaagcaatgtgcaactgacaagaaatagcaaacttccttctgcctatgtcctcactcttcttccactgaagccttctctcatcagctggagctcactatctgctacagcttggaaggccttcgctttccagaccaaactgactcaggtgacaggaatcacagctgacagctacagatcagcacaacagctgctctccagtccttccagccgctgcatcgaggtgtctaaaagagacaaagctatggcatgtggtgagggtgcttataaaaaacaaaactctcaggattcattcagagcaatcccagtgatgttacagatctaattagctaaactaaaaaaacaggggttttctccttatttctgcagttgtgattacacatggctggcaaaatggctgaaatgctattgatagtgttgcttttaaactatacaggtgttcagtcttagtttacaatgttttgaagcaggtaagtgctttgaaattacaatgatgaagagttttagcatcaaggtttgatttgtacctagtaatcagtgtgtctgccttagtagtactgactaaaaaaatttttttttgaattctgttagaattcaaatttgctgtttgacttttgaattcaatgcactgtgccacaagcctgaccgcgctatgttatgtacatttaatgtgtactcaaggaggaaaaaattactagcactactgaaaatattgcaaaattgccatagttaccgcttagagatactagttttcttctcttctttcttaaagtatatattacaactcttccataacttaatgcaaacaaagtaaattcatttcttctcacatcttaaagcaaagatatctttgtttacatgcgagaataatattctataataataccctggccctatgagccagtactttatattaggacataataataaaatgatgatatagaaagaaccagagagacctacacactgctattgatgcaaaaatccatttggaagttttctcttgtaaagggtatctaagaaagagaatagggctgaggggtgaaatgactttagaagtgggctcctatttactaagaaaaaaaccaaagccattctattgcaagatacagatcaaaggttaaaaggcaaattatactacatttagagaataaagatgtagtaattgtcaacccttaatacggcacatatgcaagtgtgctaacacaatttgcactggccataggaaaaaagcactatggaaaaaccactgactaaaaatgactgaaaaaccccgtttccctgtttcagtctaatcatttggcatctccgaatgtggtacagatttagacttgaaccaccaaagaacatcacgctgtcttatgtcaaatgctcgacaatacctctcagtaggacgttgttgcaaggctagctaattttaaatctggtatgagtaatacagtcaaacctagttagtatgcgagaaagtcgttgctaacgcatggtgagaggatgtgacgtcacagcatgagcagtccctggttgtcccattgtcagataaacgtagtgcatagatccaagtttctattccaggtctctgaaccccaaagccaggcctttcacttttgctgggtggcctggaaggccttcagctccacctggtaccactcaggggcttcaggcccactcttcccgggggggctgtggtcatagccataggcaacggtgagctcttcatcggcctccactgctctcagggtgcggatgcatttgatgggcccaaaacgggggtggacaaacatatcgtagatgcagtttggagtgaaggagtgatttgccttgtgtcccaaggaggcacagtacttggatacgtggttatagggctcaggcacatcaatgaccgtttcttcatcaagggagagggtgttcccattaagggcccagtccctgctgtcaacctcttggtgtgtaattcgaactccattataaaaagacataacagtattaggtcccacagctacctttgaaaaaagtccttctccagcactggaaataagagattcagcaacataaaccctttctgattcataaggatctggaagaagagcattggtagaaatgcaagatgaagtcgacttatcaaagtggtacactgaatttccaggcatcagttcaaagtgaggcctcccttcttcagtggacataagggtagccagtttgccttctatcatctctccatcaataaatttcccataaagtgcggtcctctcatcagggtacacataggctatcttctctccagtcatctccccatcttcatttacttctcctacaaggcttcctccatcctgatgggagaaactgggtaatatatccagcacactccatgacgaatgttatctttatactgccccttgaagatcagtctcccatctgtgtcatatt

SEQ ID NO: 16802 - RNA, 3637 nt, Homo sapiens
  source 1..3637: mol_type = other RNA
taccattagaagagctggaagacacagagagtatgaagagagttgggaggaagacatggtgaggctcagcgtggatgcattgcttcctctgatttgcgtggaggtcacagacacactgctgagttttaagctcagagtgttaccattcaatatctcatctgaagaactgattagcagactaatcactacttacaactcttcaattccttctatccaatgttgaaaaaaattccatttgaatgggataattagagtagcccccacttaggacgtaaattgtaccccactgcagccaggaccagaatgctatcactctcaggaatgaaatcattcagagcatagctgcatcgggggcatgaccagcactatcctctccctgaccgtattccctgacctggctgcacaacccacttgatcgaggttaatgcaagccatctttctcctgaagacagtcactccctttgggcacatttaaattaaagcacctatcagaatgcaagtccagaggccctggcccatccgtcacagtgtatagaacggtctctttctacagagtaagagtgaccctatcctggtgcctttaaatctaaaaactattcagttcctttggtgggcaatcttcctggaagcactgacaacttcctctcatgggtgaaccattggcttaagctttcaagcagggatccaactggatctccctgaaaccactgccacctagctgcaaagcatgcaaccgggtgctctaggaagcctggtgttgcaaagaagggaagggcaactctgtcaatgtgcccaagggccacctgaaatgaaagtcatgagcagcctgggattaagcacttttgttgtagtcttcataaagcaatgtgcaactgacaagaaatagcaaacttccttctgcctatgtcctcactcttcttccactgaagccttctctcatcagctggagctcactatctgctacagcttggaaggccttcgctttccagaccaaactgactcaggtgacaggaatcacagctgacagctacagatcagcacaacagctgctctccagtccttccagccgctgcatcgaggtgtctaaaagagacaaagctatggcatgtggtgagggtgcttataaaaaacaaaactctcaggattcattcagagcaatcccagtgatgttacagatctaattagctaaactaaaaaaacaggggttttctccttatttctgcagttgtgattacacatggctggcaaaatggctgaaatgctattgatagtgttgcttttaaactatacaggtgttcagtcttagtttacaatgttttgaagcaggtaagtgctttgaaattacaatgatgaagagttttagcatcaaggtttgatttgtacctagtaatcagtgtgtctgccttagtagtactgactaaaaaaatttttttttgaattctgttagaattcaaatttgctgtttgacttttgaattcaatgcactgtgccacaagcctgaccgcgctatgttatgtacatttaatgtgtactcaaggaggaaaaaattactagcactactgaaaatattgcaaaattgccatagttaccgcttagagatactagttttcttctcttctttcttaaagtatatattacaactcttccataacttaatgcaaacaaagtaaattcatttcttctcacatcttaaagcaaagatatctttgtttacatgcgagaataatattctataataataccctggccctatgagccagtactttatattaggacataataataaaatgatgatatagaaagaaccagagagacctacacactgctattgatgcaaaaatccatttggaagttttctcttgtaaagggtatctaagaaagagaatagggctgaggggtgaaatgactttagaagtgggctcctatttactaagaaaaaaaccaaagccattctattgcaagatacagatcaaaggttaaaaggcaaattatactacatttagagaataaagatgtagtaattgtcaacccttaatacggcacatatgcaagtgtgctaacacaatttgcactggccataggaaaaaagcactatggaaaaaccactgactaaaaatgactgaaaaaccccgtttccctgtttcagtctaatcatttggcatctccgaatgtggtacagatttagacttgaaccaccaaagaacatcacgctgtcttatgtcaaatgctcgacaatacctctcagtaggacgttgttgcaaggctagctaattttaaatctggtatgagtaatacagtcaaacctagttagtatgcgagaaagtcgttgctaacgcatggtgagaggatgtgacgtcacagcatgagcagtccctggttgtcccattgtcagataaacgtagtgcatagatccaagtttctattccaggtctctgaaccccaaagccaggcctttcacttttgctgggtggcctggaaggccttcagctccacctggtaccactcaggggcttcaggcccactcttcccgggggggctgtggtcatagccataggcaacggtgagctcttcatcggcctccactgctctcagggtgcggatgcatttgatgggcccaaaacgggggtggacaaacatatcgtagatgcagtttggagtgaaggagtgatttgccttgtgtcccaaggaggcacagtacttggatacgtggttatagggctcaggcacatcaatgaccgtttcttcatcaagggagagggtgttcccattaagggcccagtccctgctgtcaacctcttggtgtgtaattcgaactccattataaaaagacataacagtattaggtcccacagctacctttgaaaaaagtccttctccagcactggaaataagagattcagcaacataaaccctttctgattcataaggatctggaagaagagcattggtagaaatgcaagatgaagtcgacttatcaaagtggtacactgaatttccaggcatcagttcaaagtgaggcctcccttcttcagtggacataagggtagccagtttgccttctatcatctctccatcaataaatttcccataaagtgcggtcctctcatcagggtacacataggctatcttctctccagtcatctccccatcttcatttacttctcctacaaggcttcctccatctgggtaatatatccagcacactccatgacgaatgttatctttatactgccccttgaagatcagtctcccatctgtgtcatattcctgggctggaccgttcagctctccgtctacatacgtgccctggagaactcccccatcttcgtaagtgtaaactccctggccctgcaaggcatcatccacataatacccctccagggtgctgccatcaaagaagaagaacttcccccgtccgttcttttctccgtgaacaaagttcccctcaaatctgtctgtggaggagtaggtgactgtgcagaacccgtgcggtaatccgtcatcgtccaggtgcccttccaccgcctcctccaccatctcgtcgtcgctatccatggcggctggggacactgcccagctcggggctgcgcggctgcctcccgtccctctgggtgctcccggcggctgagcgagctct

SEQ ID NO: 16803 - RNA, 3123 nt, Homo sapiens
  source 1..3123: mol_type = other RNA
taccattagaagagctggaagatgtggctgtctctgagcaagtctatcttcccagccatttcttggacctgggagctcaggtggtaatgcgttgccctctgcgagttcgaggaggtggacagtctcactgtcacggtgtcatttaatcttttactgctgaggtcttgtgagtgtcttactgcaagcactccaaagtccacttgtatcagatgtttcacgttcccacacatcttcaggagactatcaacacatcttttctctttctttagaagtaacagttcctcccttctccaatccagtgcttcctccacagcacattgttcatcctggggtgaaagacttttttccctcagttgccagatgtcaagaaactgattcttgtgctttataatcagctccagttgtccaactaaaatcgtgccacttaggaggtcaccaacaactttcgtcaacacagagtcggcaacagctatcagcctcttggcatcctctgtgacatttgctagtattttctcgtcggttccacacaatctgaagacgtgcttgacatctgccaacgtgagcagatgctttaaaatgtcatcgaagttgtccgcggtcctaggccaggacttagtgatcacagcagacaagacgatgccaaatttccgcaaatcagagtaagagaacccctgaaggatactggtctgagactggcaggctgagctcacggcttcaatgatgcatttctcgaaggtcttggccacactgtcctctaagcctttggtgtcccagcaactattgcagtaggcagtgatctgggagaggggttcctcctttgtgagcctccattccatgtctcccagcaacgactccttccagccatgctccgcggggaattggatttccaccagccgcctccagacctcaatttccttgacgtatgtgaatgaggcacctgaagatgtgagcatgttctttgtaaaaacttctcggagccaccttttcgtagcagcaagggtcccttggaagactgtttggactgaattatttccagtttcatctctctgtcctgcagaatccaccagagatagaagtctaatcattctgcagacaatctcggcagataaggctggcagctcgtaaaacttaagtagctttgtgctgctgcagatggcttcatgcagtttcagacacacagtcaggtaggatggtgacaaggcctcctcgggaatcttgtcccggtaagtgtccaggagtcgcaacagcatttctaaaatgttctgaacgttctgaacatcctgaacatcctgcgtattcaagacttgctcaagtcccggaagccggtagtaaatccctgaaagacagtccaggatatgagcaggaaaacgacccaggtgctcaatgaagttttccatatacataaccaggtgactcagaggtagcagactaaaccaggaccggaagagaggctcgtctatgctcagcaaatgctgcttctctctcataaactgaagtagggaactcgtatctagcatttgttcccggaacggtgagaaggagagtccctccagagcggcccaggtgtcctcaggctgtctccaggcatccttgtgccgcggggccagctccatacagcagtgcaggacaggcagggcgcccagccaggtgtacgtccttgtgtccatgcatctttggcacaggttcaccaggtacagccgccagctctgaggtatcccaaggatgtggcttaggtcacggtgaaactcatctggtgagctggcatctgaggttaggaggtgacacaaccagtccaggctgccttctaataaaagctcaattttttccactacaaaaaggacaatcaggcctgttttcagtttactcctcactgggcagtccacaggcaaaaagtccgtgctttttccgtccggcaatggtaccacgtgttttttcagatgttgccacaggtatctcttcacctctttctccctgtactgcaaatcggtccacagctgtgcctgtccttcataaatcataggctgttgcaggacaaagcaaaactgctcgaactgggtgaagaagctgttcaggttgatggtgtcccaggtctgcaggatgctgaaggtgctgtccagcatgagcgcagcggcaatctgcttccccttcaccaggtccttcctcggcccgtctgtgatgtggttcatgactttctggagtctcccatgaggcttcatataaactatgtcatagtactgatgccagtctcctgagcccagaagtgaagattttatgaacagacagcggttgacgtactcgcccttcttctgctggtgcttgtaaatgaactcatactcaaaagattccccattataaatgacgtacttgtaaggaatgtatttatctaggtgcttcttggaaatgcagacaatgccttcaacaagaacgcggtcatgacccaagtctctggtgtagtgcagctcacagatattgctgtcccattttgactccccaaattcttctcctcctctgatgaagactttatggaggtcaggattgaatgggaaatgaagagagatgatggcgtggaagaacacggtgactcctccacccgggctcagcgtgcttgccttcacttcctggacatctgcttcctggtttttttgctccttctcgtttttcacagcagctgcacttctgttcttcccctctggcttcttgaggtcttcaggctccccttgttcattcttaccgactttttcttcagcagcagccatctcgtccttggtcttggtctcagcttccgctgaagtcggtttcctgactctctctccgctggaatgtgagcaccccgaaggccagagctttgtctgaatcatggctatatccccagcacttaaatatttgctgaataattaaatgaaagaggcgcagccgtgggcaggagagggcctcctggagccggcaggcaggaaggagacgcacctggcagtgtgttttgaaaggaggagtggttgctggtggctgtttcattctctgggtcttctctttcatttccttcccggcccctttaactgcattggctggctcagctacagcatcaactgccatagaggctgaggcccctgcctgttgctcggtggt

SEQ ID NO: 16804 - RNA, 4341 nt, Homo sapiens
  source 1..4341: mol_type = other RNA
taccattagaagagctggaagatgtggctgtctctgagcaagtctatcttcccagccatttcttggacctgggagctcaggtggtaatgcgttgccctctgcgagttcgaggaggtggacagtctcactgtcacggtgtcatttaatcttttactgctgaggtcttgtgagtgtcttactgcaagcactccaaagtccacttgtatcagatgtttcacgttcccacacatcttcaggagactatcaacacatcttttctctttctttagaagtaacagttcctcccttctccaatccagtgcttcctccacagcacattgttcatcctggggtgaaagacttttttccctcagttgccagatgtcaagaaactgattcttgtgctttataatcagctccagttgtccaactaaaatcgtgccacttaggaggtcaccaacaactttcgtcaacacagagtcggcaacagctatcagcctcttggcatcctctgtgacatttgctagtattttctcgtcggttccacacaatctgaagacgtgcttgacatctgccaacgtgagcagatgctttaaaatgtcatcgaagttgtccgcggtcctaggccaggacttagtgatcacagcagacaagacgatgccaaatttccgcaaatcagagtaagagaacccctgaaggatactggtctgagactggcaggctgagctcacggcttcaatgatgcatttctcgaaggtcttggccacactgtcctctaagcctttggtgtcccagcaactattgcagtaggcagtgatctgggagaggggttcctcctttgtgagcctccattccatgtctcccagcaacgactccttccagccatgctccgcggggaattggatttccaccagccgcctccagacctcaatttccttgacgtatgtgaatgaggcacctgaagatgtgagcatgttctttgtaaaaacttctcggagccaccttttcgtagcagcaagggtcccttggaagactgtttggactgaattatttccagtttcatctctctgtcctgcagaatccaccagagatagaagtctaatcattctgcagacaatctcggcagataaggctggcagctcgtaaaacttaagtagctttgtgctgctgcagatggcttcatgcagtttcagacacacagtcaggtaggatggtgacaaggcctcctcgggaatcttgtcccggtaagtgtccaggagtcgcaacagcatttctaaaatgttctgaacgttctgaacatcctgaacatcctgcgtattcaagacttgctcaagtcccggaagccggtagtaaatccctgaaagacagtccaggatatgagcaggaaaacgacccaggtgctcaatgaagttttccatatacataaccaggtgactcagaggtagcagactaaaccaggaccggaagagaggctcgtctatgctcagcaaatgctgcttctctctcataaactgaagtagggaactcgtatctagcatttgttcccggaacggtgagaaggagagtccctccagagcggcccaggtgtcctcaggctgtctccaggcatccttgtgccgcggggccagctccatacagcagtgcaggacaggcagggcgcccagccaggtgtacgtccttgtgtccatgcatctttggcacaggttcaccaggtacagccgccagctctgaggtatcccaaggatgtggcttaggtcacggtgaaactcatctggtgagctggcatctgaggttaggaggtgacacaaccagtccaggctgccttctaataaaagctcaattttttccactacaaaaaggacaatcaggcctgttttcagtttactcctcactgggcagtccacaggcaaaaagtccgtgctttttccgtccggcaatggtaccacgtgttttttcagatgttgccacaggtatctcttcacctctttctccctgtactgcaaatcggtccacagctgtgcctgtccttcataaatcataggctgttgcaggacaaagcaaaactgctcgaactgggtgaagaagctgttcaggttgatggtgtcccaggtctgcaggatgctgaaggtgctgtccagcatgagcgcagcggcaatctgcttccccttcaccaggtccttcctcggcccgtctgtgatgtggttcatgactttctggagtctcccatgaggcttcatataaactatgtcatagtactgatgccagtctcctgagcccagaagtgaagattttatgaacagacagcggttgacgtactcgcccttcttctgctggtgcttgtaaatgaactcatactcaaaagattccccattataaatgacgtacttgtaaggaatgtatttatctaggtgcttcttggaaatgcagacaatgccttcaacaagaacgcggtcatgacccaagtctctggtgtagtgcagctcacagatattgctgtcccattttgactccccaaattcttctcctcctctgatgaagactttatggaggtcaggattgaatgggaaatgaagagagatgatggcgtggaagaacacggtgactcctccacccgggctcagcgtgcttgccttcacttcctggacatctgcttcctggtttttttgctccttctcgtttttcacagcagctgcacttctgttcttcccctctggcttcttgaggtcttcaggctccccttgttcattcttaccgactttttcttcagcagcagccatctcgtccttggtcttggtctcagcttcctggcagtgtgttttgaaaggaggagtggttgctggtggctgtttcattctctgggtcttctctttcatttccttcccggcccctttaactgcattggctggctcagctacagcatcaactgccatagaggctgaggcccctgcctgttgctcggtggtctgcagttctgtcccgggctcagagctgcctccttttgactcaggcaacaggagctcctgggcagcatcttcagtcctagaatggccttcaccagcagaggtggggggaccggtcccctcctgggacaggcctctgcccccagaggggatggaagcgtcctggtcctccccttccgtgtggtcctggaattgcgggctgctctgagcctcacttcctgtggccactcctgcctctcccaaagcctgggcctgcagggggctgtcgccaacctcggtgggcgcggagaggccgtcaccctccagtggcgtggtggctgtgcctgggggctggctcggctggccagtggggccactctgctgggcttggctgtggggcagggctgtgtcctgaggccacgggtttgaaagcaaagtcaggtgacaggggctggcaggagaaaggggcaaggaagccagctctgaggaagcggacttgttccccttctttttcttcttccttttcttctttttgctctgctcacagtctgcagaaggcacgctggcggcctcaagcggggctgcatcctgcttccttctcttgctgggtatggcattagcagcttcccattcatcggatatgaggtctacagcagcatctaccaaaacctctgatgtagctccttcttggacggtccaggaggctttggaacagggctcctcggggttttcttgccaactgtctgagcccgggaacaagcacgggcccccttcctccttcagctcctgcccacactccatttcaccctccgaggccgacgccattgtggagttattgttctcagaatctgctatgggggctgcaggaggcagcctctctccgcactggctgcagaacttgggggtttcctccttggagacatgctggcacgaaggacactccatgggtcctgctgggactgccctgcagatccagaagcaagagcaggagtcgctggcagcctgctatatactacatgtcctgtcacgtgaccacggcttcagtttcattttcctggccttgagccccgcgctcgggcgacttcgccaagtcggaaggacgctgcgcggtgcggttcagacggggcgatgcctccctcgtaaaagttaggagtctgtttttgcaacttcacttttccgttgttgccattcgtacaggcgcaggattcccgggcggacctgcaggcccgggtccggctgtccccttccactacaccccccgtgccccggccacttcccgggggcagcactgccggggcgcaaagcctcctccgcgctctgcgctccggggatgtcgccggggtcccaggcgtgcccgctgcccccaccccgacccctcccgcagccggggaacagggtcagtgggcgccgcgggcggggctgg

SEQ ID NO: 16805 - RNA, 4054 nt, Homo sapiens
  source 1..4054: mol_type = other RNA
taccattagaagagctggaagatgtggctgtctctgagcaagtctatcttcccagccatttcttggacctgggagctcaggtggtaatgcgttgccctctgcgagttcgaggaggtggacagtctcactgtcacggtgtcatttaatcttttactgctgaggtcttgtgagtgtcttactgcaagcactccaaagtccacttgtatcagatgtttcacgttcccacacatcttcaggagactatcaacacatcttttctctttctttagaagtaacagttcctcccttctccaatccagtgcttcctccacagcacattgttcatcctggggtgaaagacttttttccctcagttgccagatgtcaagaaactgattcttgtgctttataatcagctccagttgtccaactaaaatcgtgccacttaggaggtcaccaacaactttcgtcaacacagagtcggcaacagctatcagcctcttggcatcctctgtgacatttgctagtattttctcgtcggttccacacaatctgaagacgtgcttgacatctgccaacgtgagcagatgctttaaaatgtcatcgaagttgtccgcggtcctaggccaggacttagtgatcacagcagacaagacgatgccaaatttccgcaaatcagagtaagagaacccctgaaggatactggtctgagactggcaggctgagctcacggcttcaatgatgcatttctcgaaggtcttggccacactgtcctctaagcctttggtgtcccagcaactattgcagtaggcagtgatctgggagaggggttcctcctttgtgagcctccattccatgtctcccagcaacgactccttccagccatgctccgcggggaattggatttccaccagccgcctccagacctcaatttccttgacgtatgtgaatgaggcacctgaagatgtgagcatgttctttgtaaaaacttctcggagccaccttttcgtagcagcaagggtcccttggaagactgtttggactgaattatttccagtttcatctctctgtcctgcagaatccaccagagatagaagtctaatcattctgcagacaatctcggcagataaggctggcagctcgtaaaacttaagtagctttgtgctgctgcagatggcttcatgcagtttcagacacacagtcaggtaggatggtgacaaggcctcctcgggaatcttgtcccggtaagtgtccaggagtcgcaacagcatttctaaaatgttctgaacgttctgaacatcctgaacatcctgcgtattcaagacttgctcaagtcccggaagccggtagtaaatccctgaaagacagtccaggatatgagcaggaaaacgacccaggtgctcaatgaagttttccatatacataaccaggtgactcagaggtagcagactaaaccaggaccggaagagaggctcgtctatgctcagcaaatgctgcttctctctcataaactgaagtagggaactcgtatctagcatttgttcccggaacggtgagaaggagagtccctccagagcggcccaggtgtcctcaggctgtctccaggcatccttgtgccgcggggccagctccatacagcagtgcaggacaggcagggcgcccagccaggtgtacgtccttgtgtccatgcatctttggcacaggttcaccaggtacagccgccagctctgaggtatcccaaggatgtggcttaggtcacggtgaaactcatctggtgagctggcatctgaggttaggaggtgacacaaccagtccaggctgccttctaataaaagctcaattttttccactacaaaaaggacaatcaggcctgttttcagtttactcctcactgggcagtccacaggcaaaaagtccgtgctttttccgtccggcaatggtaccacgtgttttttcagatgttgccacaggtatctcttcacctctttctccctgtactgcaaatcggtccacagctgtgcctgtccttcataaatcataggctgttgcaggacaaagcaaaactgctcgaactgggtgaagaagctgttcaggttgatggtgtcccaggtctgcaggatgctgaaggtgctgtccagcatgagcgcagcggcaatctgcttccccttcaccaggtccttcctcggcccgtctgtgatgtggttcatgactttctggagtctcccatgaggcttcatataaactatgtcatagtactgatgccagtctcctgagcccagaagtgaagattttatgaacagacagcggttgacgtactcgcccttcttctgctggtgcttgtaaatgaactcatactcaaaagattccccattataaatgacgtacttgtaaggaatgtatttatctaggtgcttcttggaaatgcagacaatgccttcaacaagaacgcggtcatgacccaagtctctggtgtagtgcagctcacagatattgctgtcccattttgactccccaaattcttctcctcctctgatgaagactttatggaggtcaggattgaatgggaaatgaagagagatgatggcgtggaagaacacggtgactcctccacccgggctcagcgtgcttgccttcacttcctggacatctgcttcctggtttttttgctccttctcgtttttcacagcagctgcacttctgttcttcccctctggcttcttgaggtcttcaggctccccttgttcattcttaccgactttttcttcagcagcagccatctcgtccttggtcttggtctcagcttcctggcagtgtgttttgaaaggaggagtggttgctggtggctgtttcattctctgggtcttctctttcatttccttcccggcccctttaactgcattggctggctcagctacagcatcaactgccatagaggctgaggcccctgcctgttgctcggtggtctgcagttctgtcccgggctcagagctgcctccttttgactcaggcaacaggagctcctgggcagcatcttcagtcctagaatggccttcaccagcagaggtggggggaccggtcccctcctgggacaggcctctgcccccagaggggatggaagcgtcctggtcctccccttccgtgtggtcctggaattgcgggctgctctgagcctcacttcctgtggccactcctgcctctcccaaagcctgggcctgcagggggctgtcgccaacctcggtgggcgcggagaggccgtcaccctccagtggcgtggtggctgtgcctgggggctggctcggctggccagtggggccactctgctgggcttggctgtggggcagggctgtgtcctgaggccacgggtttgaaagcaaagtcaggtgacaggggctggcaggagaaaggggcaaggaagccagctctgaggaagcggacttgttccccttctttttcttcttccttttcttctttttgctctgctcacagtctgcagaaggcacgctggcggcctcaagcggggctgcatcctgcttccttctcttgctgggtatggcattagcagcttcccattcatcggatatgaggtctacagcagcatctaccaaaacctctgatgtagctccttcttggacggtccaggaggctttggaacagggctcctcggggttttcttgccaactgtctgagcccgggaacaagcacgggcccccttcctccttcagctcctgcccacactccatttcaccctccgaggccgacgccattgtggagttattgttctcagaatctgctatgggggctgcaggaggcagcctctctccgcactggctgcagaacttgggggtttcctccttggagacatgctggcacgaaggacactccatgggtcctgctgggactgccctgcagatccagaagcaagagcaggagtcgctggcagcctgctatatactacatgtcctgtcacgtgaccacggcttcagtttcattttctgcggcccccgagctcgccgcctgccgcgcgctgtcgcccctcgggtcacggggccctgggccccgccctgcccgccgccgc

SEQ ID NO: 16806 - RNA, 3958 nt, Homo sapiens
  source 1..3958: mol_type = other RNA
taccattagaagagctggaagatgtggctgtctctgagcaagtctatcttcccagccatttcttggacctgggagctcaggtggtaatgcgttgccctctgcgagttcgaggaggtggacagtctcactgtcacggtgtcatttaatcttttactgctgaggtcttgtgagtgtcttactgcaagcactccaaagtccacttgtatcagatgtttcacgttcccacacatcttcaggagactatcaacacatcttttctctttctttagaagtaacagttcctcccttctccaatccagtgcttcctccacagcacattgttcatcctggggtgaaagacttttttccctcagttgccagatgtcaagaaactgattcttgtgctttataatcagctccagttgtccaactaaaatcgtgccacttaggaggtcaccaacaactttcgtcaacacagagtcggcaacagctatcagcctcttggcatcctctgtgacatttgctagtattttctcgtcggttccacacaatctgaagacgtgcttgacatctgccaacgtgagcagatgctttaaaatgtcatcgaagttgtccgcggtcctaggccaggacttagtgatcacagcagacaagacgatgccaaatttccgcaaatcagagtaagagaacccctgaaggatactggtctgagactggcaggctgagctcacggcttcaatgatgcatttctcgaaggtcttggccacactgtcctctaagcctttggtgtcccagcaactattgcagtaggcagtgatctgggagaggggttcctcctttgtgagcctccattccatgtctcccagcaacgactccttccagccatgctccgcggggaattggatttccaccagccgcctccagacctcaatttccttgacgtatgtgaatgaggcacctgaagatgtgagcatgttctttgtaaaaacttctcggagccaccttttcgtagcagcaagggtcccttggaagactgtttggactgaattatttccagtttcatctctctgtcctgcagaatccaccagagatagaagtctaatcattctgcagacaatctcggcagataaggctggcagctcgtaaaacttaagtagctttgtgctgctgcagatggcttcatgcagtttcagacacacagtcaggtaggatggtgacaaggcctcctcgggaatcttgtcccggtaagtgtccaggagtcgcaacagcatttctaaaatgttctgaacgttctgaacatcctgaacatcctgcgtattcaagacttgctcaagtcccggaagccggtagtaaatccctgaaagacagtccaggatatgagcaggaaaacgacccaggtgctcaatgaagttttccatatacataaccaggtgactcagaggtagcagactaaaccaggaccggaagagaggctcgtctatgctcagcaaatgctgcttctctctcataaactgaagtagggaactcgtatctagcatttgttcccggaacggtgagaaggagagtccctccagagcggcccaggtgtcctcaggctgtctccaggcatccttgtgccgcggggccagctccatacagcagtgcaggacaggcagggcgcccagccaggtgtacgtccttgtgtccatgcatctttggcacaggttcaccaggtacagccgccagctctgaggtatcccaaggatgtggcttaggtcacggtgaaactcatctggtgagctggcatctgaggttaggaggtgacacaaccagtccaggctgccttctaataaaagctcaattttttccactacaaaaaggacaatcaggcctgttttcagtttactcctcactgggcagtccacaggcaaaaagtccgtgctttttccgtccggcaatggtaccacgtgttttttcagatgttgccacaggtatctcttcacctctttctccctgtactgcaaatcggtccacagctgtgcctgtccttcataaatcataggctgttgcaggacaaagcaaaactgctcgaactgggtgaagaagctgttcaggttgatggtgtcccaggtctgcaggatgctgaaggtgctgtccagcatgagcgcagcggcaatctgcttccccttcaccaggtccttcctcggcccgtctgtgatgtggttcatgactttctggagtctcccatgaggcttcatataaactatgtcatagtactgatgccagtctcctgagcccagaagtgaagattttatgaacagacagcggttgacgtactcgcccttcttctgctggtgcttgtaaatgaactcatactcaaaagattccccattataaatgacgtacttgtaaggaatgtatttatctaggtgcttcttggaaatgcagacaatgccttcaacaagaacgcggtcatgacccaagtctctggtgtagtgcagctcacagatattgctgtcccattttgactccccaaattcttctcctcctctgatgaagactttatggaggtcaggattgaatgggaaatgaagagagatgatggcgtggaagaacacggtgactcctccacccgggctcagcgtgcttgccttcacttcctggacatctgcttcctggtttttttgctccttctcgtttttcacagcagctgcacttctgttcttcccctctggcttcttgaggtcttcaggctccccttgttcattcttaccgactttttcttcagcagcagccatctcgtccttggtcttggtctcagcttcctggcagtgtgttttgaaaggaggagtggttgctggtggctgtttcattctctgggtcttctctttcatttccttcccggcccctttaactgcattggctggctcagctacagcatcaactgccatagaggctgaggcccctgcctgttgctcggtggtctgcagttctgtcccgggctcagagctgcctccttttgactcaggcaacaggagctcctgggcagcatcttcagtcctagaatggccttcaccagcagaggtggggggaccggtcccctcctgggacaggcctctgcccccagaggggatggaagcgtcctggtcctccccttccgtgtggtcctggaattgcgggctgctctgagcctcacttcctgtggccactcctgcctctcccaaagcctgggcctgcagggggctgtcgccaacctcggtgggcgcggagaggccgtcaccctccagtggcgtggtggctgtgcctgggggctggctcggctggccagtggggccactctgctgggcttggctgtggggcagggctgtgtcctgaggccacgggtttgaaagcaaagtcaggtgacaggggctggcaggagaaaggggcaaggaagccagctctgaggaagcggacttgttccccttctttttcttcttccttttcttctttttgctctgctcacagtctgcagaaggcacgctggcggcctcaagcggggctgcatcctgcttccttctcttgctgggtatggcattagcagcttcccattcatcggatatgaggtctacagcagcatctaccaaaacctctgatgtagctccttcttggacggtccaggaggctttggaacagggctcctcggggttttcttgccaactgtctgagcccgggaacaagcacgggcccccttcctccttcagctcctgcccacactccatttcaccctccgaggccgacgccattgtggagttattgttctcagaatctgctatgggggctgcaggaggcagcctctctccgcactggctgcagaacttgggggtttcctccttggagacatgctggcacgaaggacactccatgggtcctgctgggactgccctgcggcccccgagctcgccgcctgccgcgcgctgtcgcccctcgggtcacggggccctgggccccgccctgcccg

SEQ ID NO: 16807 - RNA, 3875 nt, Homo sapiens
  source 1..3875: mol_type = other RNA
taccattagaagagctggaagatgtggctgtctctgagcaagtctatcttcccagccatttcttggacctgggagctcaggtggtaatgcgttgccctctgcgagttcgaggaggtggacagtctcactgtcacggtgtcatttaatcttttactgctgaggtcttgtgagtgtcttactgcaagcactccaaagtccacttgtatcagatgtttcacgttcccacacatcttcaggagactatcaacacatcttttctctttctttagaagtaacagttcctcccttctccaatccagtgcttcctccacagcacattgttcatcctggggtgaaagacttttttccctcagttgccagatgtcaagaaactgattcttgtgctttataatcagctccagttgtccaactaaaatcgtgccacttaggaggtcaccaacaactttcgtcaacacagagtcggcaacagctatcagcctcttggcatcctctgtgacatttgctagtattttctcgtcggttccacacaatctgaagacgtgcttgacatctgccaacgtgagcagatgctttaaaatgtcatcgaagttgtccgcggtcctaggccaggacttagtgatcacagcagacaagacgatgccaaatttccgcaaatcagagtaagagaacccctgaaggatactggtctgagactggcaggctgagctcacggcttcaatgatgcatttctcgaaggtcttggccacactgtcctctaagcctttggtgtcccagcaactattgcagtaggcagtgatctgggagaggggttcctcctttgtgagcctccattccatgtctcccagcaacgactccttccagccatgctccgcggggaattggatttccaccagccgcctccagacctcaatttccttgacgtatgtgaatgaggcacctgaagatgtgagcatgttctttgtaaaaacttctcggagccaccttttcgtagcagcaagggtcccttggaagactgtttggactgaattatttccagtttcatctctctgtcctgcagaatccaccagagatagaagtctaatcattctgcagacaatctcggcagataaggctggcagctcgtaaaacttaagtagctttgtgctgctgcagatggcttcatgcagtttcagacacacagtcaggtaggatggtgacaaggcctcctcgggaatcttgtcccggtaagtgtccaggagtcgcaacagcatttctaaaatgttctgaacgttctgaacatcctgaacatcctgcgtattcaagacttgctcaagtcccggaagccggtagtaaatccctgaaagacagtccaggatatgagcaggaaaacgacccaggtgctcaatgaagttttccatatacataaccaggtgactcagaggtagcagactaaaccaggaccggaagagaggctcgtctatgctcagcaaatgctgcttctctctcataaactgaagtagggaactcgtatctagcatttgttcccggaacggtgagaaggagagtccctccagagcggcccaggtgtcctcaggctgtctccaggcatccttgtgccgcggggccagctccatacagcagtgcaggacaggcagggcgcccagccaggtgtacgtccttgtgtccatgcatctttggcacaggttcaccaggtacagccgccagctctgaggtatcccaaggatgtggcttaggtcacggtgaaactcatctggtgagctggcatctgaggttaggaggtgacacaaccagtccaggctgccttctaataaaagctcaattttttccactacaaaaaggacaatcaggcctgttttcagtttactcctcactgggcagtccacaggcaaaaagtccgtgctttttccgtccggcaatggtaccacgtgttttttcagatgttgccacaggtatctcttcacctctttctccctgtactgcaaatcggtccacagctgtgcctgtccttcataaatcataggctgttgcaggacaaagcaaaactgctcgaactgggtgaagaagctgttcaggttgatggtgtcccaggtctgcaggatgctgaaggtgctgtccagcatgagcgcagcggcaatctgcttccccttcaccaggtccttcctcggcccgtctgtgatgtggttcatgactttctggagtctcccatgaggcttcatataaactatgtcatagtactgatgccagtctcctgagcccagaagtgaagattttatgaacagacagcggttgacgtactcgcccttcttctgctggtgcttgtaaatgaactcatactcaaaagattccccattataaatgacgtacttgtaaggaatgtatttatctaggtgcttcttggaaatgcagacaatgccttcaacaagaacgcggtcatgacccaagtctctggtgtagtgcagctcacagatattgctgtcccattttgactccccaaattcttctcctcctctgatgaagactttatggaggtcaggattgaatgggaaatgaagagagatgatggcgtggaagaacacggtgactcctccacccgggctcagcgtgcttgccttcacttcctggacatctgcttcctggtttttttgctccttctcgtttttcacagcagctgcacttctgttcttcccctctggcttcttgaggtcttcaggctccccttgttcattcttaccgactttttcttcagcagcagccatctcgtccttggtcttggtctcagcttcctggcagtgtgttttgaaaggaggagtggttgctggtggctgtttcattctctgggtcttctctttcatttccttcccggcccctttaactgcattggctggctcagctacagcatcaactgccatagaggctgaggcccctgcctgttgctcggtggtctgcagttctgtcccgggctcagagctgcctccttttgactcaggcaacaggagctcctgggcagcatcttcagtcctagaatggccttcaccagcagaggtggggggaccggtcccctcctgggacaggcctctgcccccagaggggatggaagcgtcctggtcctccccttccgtgtggtcctggaattgcgggctgctctgagcctcacttcctgtggccactcctgcctctcccaaagcctgggcctgcagggggctgtcgccaacctcggtgggcgcggagaggccgtcaccctccagtggcgtggtggctgtgcctgggggctggctcggctggccagtggggccactctgctgggcttggctgtggggcagggctgtgtcctgaggccacgggtttgaaagcaaagtcaggtgacaggggctggcaggagaaaggggcaaggaagccagctctgaggaagcggacttgttccccttctttttcttcttccttttcttctttttgctttcttggacggtccaggaggctttggaacagggctcctcggggttttcttgccaactgtctgagcccgggaacaagcacgggcccccttcctccttcagctcctgcccacactccatttcaccctccgaggccgacgccattgtggagttattgttctcagaatctgctatgggggctgcaggaggcagcctctctccgcactggctgcagaacttgggggtttcctccttggagacatgctggcacgaaggacactccatgggtcctgctgggactgccctgcagatccagaagcaagagcaggagtcgctggcagcctgctatatactacatgtcctgtcacgtgaccacggcttcagtttcattttctgcggcccccgagctcgccgcctgccgcgcgctgtcgcccctcgggtcac

SEQ ID NO: 16808 - RNA, 2520 nt, Homo sapiens
  source 1..2520: mol_type = other RNA
tacccagagcatgcagtgtgaaattttgcaatctatcccaaacaatatactgcataggcatcgtctttaaatacacacattttctgtttccaagtactacagataactcataattcctataaaaaattacacaatttaatcaagatggtagtacgtggagattatttccttttagtttattgtttaaatacatgtcttgccaatcacaaaatatctagtgtagccaaagacataagaaatccctgtatgaatcaaaaagtgccattcttgcagctttctgtcacaaggatgctgagaaatgtactgtaacagtttaggaaacacaagattgtctcaattttaagtttcaatcattaatcctcttcagaactggaatcaccctcttggtcagaaagttcgggaacagggaagcggagaatggcagctaccccagtcaactggctgagctgttccccagaaacgtgaagactagagaatatcctaacggtgcctgcattctctttcacactgtccaccagcctcacataccggctccgtgtggctacatcctgatgcctgaagagctcatcgctgatgagcaatgtgtcaattgccatggcttcattggccttctccacctgcttgagtccatagaaagctcgatccggttcatgctgtaacattttatagaagtcatccaaggctttgacttccccagcagctttagtgtctgaaaggcggctagccacagtagggtcacaaagggcctctttcagggagtacttgtgtccggaggaggcatgtacctgaagaaatttggaccggttttccaggagcagtttgttgtcggtcttcactgcttgttgaaacaggtagtcgcagaactgctccctcacaaatcctgggctggccaccaggatgcactttacaacatcaaagtgtatgtggcgctggatagcctggaccacctgttcatagaaccgctccaaggcccggtcatgctgagagcaattgcctttccttttcctagggatgttcacctccaccttggcccgagtgagggtcatgctgggagtgactaagcagatatgggcgaggccttcctgcatgaccacagccgccacatcagcgctccaggctgggtcacaggcctgctcgatgcgctccagtaccacactatcccactgcttcttggccagggtgaactggcggttgggctccagctcgatggtgtggtaagcccccatcttgacatactcattctcttggatgttggtccccttaacccgcagctggcaggcttgagagtcgaagtcgatggcctccacgcagagagtgagggtagtgcggacccggttgctgcccacgctgcccgtggaggactctgtctgtaccttgcggatggtggaggcgcgcaggctgtcgcccacctgcacgaggttgtaagtgtgccacatgtcctcaggctcctcggggaccagggtcacctggcccgcattgtccttctcgatgttcttcctcacgagcttcatggccaaggaaggggctcactgacagaaccaaaggaaccaaggaggtcctcacctccgccccgggagaggggatgggaatgcaggccaggaagggggcggggcccggtttctaagggcacttgcctggcgggaaggaaacacgcttgcttcgactcatgcagcctagggcagcacttcctctatcctttcctctctcagtctcccggcgcgctgcgtctaacaggctcggggaacactgcagcgaaaatctacccctacacagttcccgctggcagcacgcaacagcgggctgacgaaatgaaggcgcatgcgcagcccccgtcccgcgacccgacgcacgtctcccgtccccaaaggagaggcggggccgcagttcgcgcgtgcgcaggcgcactaagctgtgaggcgctccggacgaatgaactccctcaagaaggtgcacagagtggtggcgagtcctttattttaatgccaaacttcaacttcctaagttttctcttccatccctgtcagtgaggagccagcagcaggcgacagcgacccctgggcgggcgcggggccgaggggccatggccggagcagcctcagcgccagggggccgcgctggttcgcagggcaggaccgggcgcgggagctgcgctctctggctgggccacttatcccgctgccgcggttcccagtcctctgccccagtggcagcggcgcccaggagcgggagaggagtgatttcctgtgttttcgtcgaattcctctaaatgcgctccacgcttttcacatcccagacggattgccacatcgcccgccccttcgcgctcttggtctctgaaatctcactggcagcttcccaggctctgtccgagacatggacaaataaagccagcttcgcgggtccgtgtttaggctaaagtccacgggctgtagaagcaaaccttaaagggacatctgcctttcattgagagggtgatctcgttctccgggccaaatcccctaaggtggtaggaaggcgggt

SEQ ID NO: 16809 - RNA, 63 nt, Homo sapiens
  source 1..63: mol_type = other RNA
tacccagtctccggtgcagcctgttgtcaaggctgcaccggagactgggtaagacatgacaag

SEQ ID NO: 16810 - RNA, 63 nt, Homo sapiens
  source 1..63: mol_type = other RNA
tacccagtctccggtgcagccttgacaacaggctgcaccggagactgggtaagacatgacaag

SEQ ID NO: 16811 - RNA, 2050 nt, Homo sapiens
  source 1..2050: mol_type = other RNA
tacctgggagactgaggttggaggatcccttgagctcaggatgtcaaggccacagtgagctatgatcacaacagcctgagcaacagtgtaagactctgtctcaacaaaatgaataagtaaagaaataatttggaggccattctgtaaggtacttttatttgttgggatgcaagtttggctctagtaatataactcaaataacagtaacttatacaaaatggaattttattcctctcaaataacagtacaacataaacaatccatgacttatatggtggcctcaaagatgctgggttctacagttcttcacaagttttttcagttatgatttttagttctagtcatcacattttcatcttagctttgtcttggcaggctgatgaggggttgtttatgacacctcttgctaaggctaaaaagcttgtgtacaattttctgcgcctttaggaaaagttgtttcatgctgttctccagttgttcataacggcgctgaaaattagaatccattgtccacaaatgcattatagtagatgtgttgaggaaataattcataggtagccttttcataaataacttgaattcatctgattcctcaaagtcactgttgtaagctttccaggtttcagttattcgaagaagattctcttccatggcttgaatgtccatggaggggcagttgcattctggaaatttgggaccacagtgacaccagcagtcattttccttgcagataaactctccctctgaattgcaagcaatgtagctcaaagctgcttgtacaaaacgttcctgaagatagtctgggagaagtacttgaagcccttgcaactgaatcttattctcaggactctgaaccagaacagaactgacagaatctaggttgtcatagttactgcagccaagaggaccagtccgtgtttctgttacctttatggcagtggatgcaatttgaatgtggtgaagtctccgaagggtgctgtccctgtcaatgaaataagaagcggctagctgatgtagcgtctccagagtgaccgaagagctattggtggtggaatcacttccttcagctcgtttgctcaacttccgcttgtccacaaaaattgtgagtgactcctctcctcccagagtagcagatagcaagaaatgtgtcccatatttcttgataaggttttctgtgatttgctgaagggtaggtcgacgtcccaaaagtcttatgttgcggaagaattcaggggcaagaggcagaggagagccaaggaaatttcttctctcaactgcaaggttatttactttccagcggccaaactccctgtatatcttgtatcttgtgctaaatccctgccggcttctgtccacaaaatctgtgtattcctgtgagcgatggaagggtcccttatcagagaggagccagtcgaaggggcttgtggcatgctgatccgaaacagcagcaaccgctaaaacccagcaatgaagactcagtgctatccactcccatagagccatcagagagaacaattcagcaccagctctgcttcgccatatcatgcttccactggggatttagagccttcattctctcagctttccctcaacacctgcttaactgcatgatgacaaacaaatctatgtaacacgcaaaagaaagtccccaaaatctgaatcatctgtcttccaagctgctgtggcagttttatatcctggtgctctcttctttgcttacgtacatttgactagatagaatatttttaagtgatactaaggttaatttgcaaccctagtcaccttttccttctttcaaacagccagtgggcattttacacagctccaaacatgcatcttatcttcggaggtagtgcctacacggcgtttcccagcagaattcctgttacaaggaggttccttctctaaagggctgatcacgttctcgacctggtgcaaagtaaaagcctctccggttcaactcttggggactaggagaacagccatcagagacttaaactctctgtcactgtttggctgtggaaccagcagtaaccagcggccaagaagc

SEQ ID NO: 16812 - RNA, 3254 nt, Homo sapiens
  source 1..3254: mol_type = other RNA
tacggtgagcctgtcattattcagagaggctagatcctctgtgttgagaaggatcatgatgggctcctcggtgttctccaggtagcggcaccacaccatgaaggcagcccgtattggaagaatcttcatctccgcttgagagtactcaacctcgataggggagatgttgcgggagtagaaagcgcagcaggctctcttgccggtttggtcgtcgatttggatcagggaggcgtgcagggccgtgccggtgacgccggtttccaagtagaatgggttctggggcttggggtggtggaggagaggcgccttgcggaaagccctcttcaggcactcgaaggcctcttgctcctcgactccccagtagaactggtaggagctcagcagctgccgcaccaggggctctgcgatgatgctgaagcgctccacgaagtggcggtaggggaagacgaattcgatgaagtttcgcagagatagcttggagccaggggtagggtaccctgttatgatggtcatgacgttcttgttcagtttcacccctttgggggtgacgacgaagcccaggaattccacggtttggcggtggaactggctcttgtccagggagcagtagacgttgtgatggcggaagcggaccaggacttggcggacgtggtggaggtgctcctcctgactcattgagtagatcaggacttcctggccataagaaagcacaaagaaccctagcatgtcctttaggatgaagtgaatcacgttctgaggtatgatagggtctggggagagcgcaaacggctggtagctcttcatctcttcaagctccaaaccaaacgctgctttccacacatcttcggtgcggtgcccgttcacgctttcctccacaatggtcccacgcagctccagttttgtgaaccactcggctccgtgtaactggtcaaacagttccggaatcatctgtatgtagtcctgtctgttggtcagcatgtcctgcaggtcccagtattcctcctgtagcctggctctttcttgcatcctggcacccacaggttcccaaggcgcggtggagggacactcgtaaaaggtctcgctgtgatcactgtctccagcctgctgaagctcagagggctctgattcagaaagatcatcggatccgtctgagcttggctggtcggaagtctcatcatctgcttccttcgggttaaacacgtcggccaggtctgagtatgggtgtggcagtccgggtagcaggctcatgccgtgcctctctagggcaatgcatggcgggggcgggcggaagcagttcttcaggcagtagggagagtggaaggtgcagcggcctttgatccagtcgacttcgggggcgtggactcggagccagcggatgcctaggaccacagagaagttcggtgaaggtacgatgtcaaattcgatggactcctggtggttctggtggatacacaccaggggctccgtgtagagccagacaggctcgttgccaatcagcgagccgtccacggattggaccggctgtgggtacggcttctcgtagagctcgacgtagtgctcttgggcgaacttctcatccatgaagttgccgtcagctcccgaatccaccagggcctggaccgcgacgctgtggtaggggttcactctcaccatgagcagcaggaagaggtgggcgcgattgatgtccggatggacttcgctgggcaaccagctgctgaccatccacctctctggagcaggtgagtcgatccaggtcaggttccgggggcgggcctcggggggcagcctgagcatagctcttctctctgccagcttctcttctatttgcaggatgagcacaatcagactgtctagggaatccggctgagggacccggaatagatagtgcctgatctcctcgttgagcccctggcacaagtgggcctgcaggacttcatctggccagcccaagatgggtaccaggctctggaactcatcgatgtactcagtggcagagcggccgccctgcctgatggtgaacatggcctcttctgccacacgcagtgcctggcggtactcaaacacttcggacatggcctccaggaaggctgggaagtctccgatcagggggctgttttcctgcagtagagctttggcccattctaatgccaagccggacaggtgattgatgacatagccaactctcagacggtcgttatagaacattcttgggtagctctgtaaggtcagttggcagagtacgatgaactcgtggaattctctgcgatcgccagagaagtgctttggggcgggcagttggcctgcattgatccctttgatcaagatctcttctgctactctctgttgctctttgaggtcttgcattcggaagtacagcgagatgatggacctcaccatggccataagttctgcggttgagtgctcggtctggttttgctcttgaggagtctcctcccttcccgattccttcaggtcagtgtgagcctcttgttcttctcgggctcccgatgggttgactgatgcttctttcatcctatcagatgctccactgagtggatccccccttgcctggtgtgaaccgttgcatgactcctccaggtcttggagtaggtcattgggtggatcctctatttccttacgtgggccactggatggctcctccatgtcttggagtagatcagtgggcagctcttccatttcctggagtgggccactggggggctccttcttttcctgggctgggccgctggctggccctgcctctccccgcactccactgcccgacgtcgcctcggtggtgttggatgagccctcggaggactccatttgttttgatgatggattcttatgctccatcatcgtctcaaatgagtcttcagagggttctatcatttcgtcggatggaaaggagtgtattctgaagattggtaaggttgtgatggcgtccagtcagtagctgggaccgtggagatcagaaccttggctgcaagcgttcaagtggatctcctcccgtcctgtgccactcgatcctcgctgcttgcttccccgggcccagtcccaagcgtgaggctggggatgaagtgatgccggtggcttagtgatgccggtggcttcctgtcctcgaagctcagtcggtcgtctctcagctggtgtgaggctgggccaggatggaaccccagactctccgaggctccccaccacaccctgctgctgaaggctgctcagcgaggctgtgccgagtgctgggggggtgt

SEQ ID NO: 16813 - RNA, 5781 nt, Homo sapiens
  source 1..5781: mol_type = other RNA
tacgtagatatatatgtattttaaagttaaatctagggaaaaatttccacttaagttacataaaatttgatgaagaacatttgtcaaatgttaagttttagtctattctttaataacacagtgcagctcaaactgtcattgaatataagatcagttaaaaattaaggaaagtatttcaaaacaggtttctaatttgaactgggcaaacattttgatataatgttgaagctttgatatgatgttttgatatcatagtttagagggcgaggggagctgtgacaattctgttttttgcttgaaagattatcttatattctctgatttttttcctctctcgaatgtgttctaacaaggcatacacaacagtagaaaaaatatataaaagaaaggaaagtgcgtcttactaaatttaataattaatattgttgacataaaagtaaaaggcaagcttaacttttgaaggctgactcatgaagaattttttcattaatcaaacactgactacatttaagctataaaattttcacatggaatactgaaacaataatgtaccatgattctatctctaaatttattttaaatttagagctttcatattttatagttattctttaccagttcagatgtttctatatctctatatattcatatagaattatagattttatattcatgtgtaattaagtcacaaaactatgtaaaataaaattctgtgtgagtgatatgactgatgacttcttaaaatagtaatcttcaattacatattttacaccacaaaatgtacagacacccagtttttttctaacaacaaatacaggtgaatttatcgattctttataaaagctttaagtgattctaaattcaaagtcatagaaatagaatcagacttatgcagattgttagatagtttgatagtacatagtcagtgctctgtctgataacatcaatagctacatctttggcattgaaaattcaatatgagtttttgacaaaattttgtagcttagagcatcattttcttttaaacaaggaaaaacacggttgagtaagatatggaaattgggagaaaactattaatgattttttcttagtaagtttgtctttgggaccctgaattaccttttattttattgtatgatgtggactgtatgcatccatttaaaaaccaactgagttgtaccacattttaggaaaattatataatataatatatatattttatatttatttagaagctttgaaatagtacagtaaacactttgcaacacggtgtataaactacagaatgtctttgatattttgtgggtcttcagaatacaacattttttataacccacaggtgaaaagaacataatcacaatttctcttgtaaagttggaatagcttgcggaacacttgatcacacaaaaataatataaaacagtcaagtttaaaacagtgatattgcatttataatgcacaaatttcctttatctttatgactggcttctcgtggtgaatataaacatctaaagggctcagtgacatttggagagagaaagatagatagtgctgtaaacaggcacacactgatcggggaggcaaaatctgttgcctctaaagtttctacagttctgcacatttcaactcatttctcaggcctgctgagagcaattaggtcctataattggccatgatgactccatccgaaatctaatactcagttacacatgactaactggatggccaagataatgaagttgaaaagttgatgcttttgttggtcgactttgtgcaaatcatgctgcttcaggtaagtcctgtagaattgactagcatatccttttccgtgtcaaatatggtggtttgtaaggcgctcgcgtattagtcagcagtccatccagctccttcctctccagagtgctgtgaagggccttctctttgccaaaggtggaaaaggaccgctctgccccaggctgggcttctggagtttcaaacacctcagtgtctggaacagagtccatgccaggaacatgcagattgctgcgataatcagcagcctggcgtccatcagaagggacaaaagaaggcatccagcaccgatctgagtggcccagagctttacattcctcagtgcaattggagaagagatccataccagctgactgggcacggttggtggcatcatgatcactatctccctgttcactgtctccatgaccactgtccttagagcttactatgtcggcttcctggaatgcagaactgttaactcggcgaggtctgtcaactagatagctgagctctgctcgctggtgtttagtctcgttggacaaaatgcttccgttggagatgatatcaggctgctggtcggtgtaaccggtgacgatggccccgcaggggttgtgctcagtgtccgtactccgcgaagggctgcagggcttaagaaacatcaggtcggtcttggcggactcaggggtcaggcatacctgatagcagtaattctggttgtggtggtgggagccaaagcccccggactcctctatcggcacctgggccgggttactgggtacattggagctctgcaccagcatgatgtctgacttgctgagtttcttcttgcgcgcccgggcttggcggccacagcaggtcgaacctccgccaccgcagcagcagcagcagaggcagcaatcgctggccagacaagtatagatgttgagcttcttctctttttggcaacgcacggccagcacgatcatggccagcaggaagatgaaggacaccgagcccaacgcgatgatgaggatgagggtgaggtctagcgaggtttccccgccgccagagcgactggggcgctggtgctctcctgaccctccgcctccgctcccgcccccgccctggggctccacggcgccatccaccagctgaaccaccagggtggcggtggaggaaaggggcggctgcccatggtcgcgcacctcgatcaccagctcataaggccgctgggggtcgcgcttggccgggactcggcgtgctgtgcgcagctccccggtgcgccagtccatgcgaaagaggttcatttcgttgccacgcacgatgctgtaagtgagccgggcgttctcgccgtcgtccgcgtccacggcggccacgcgggtgagcaggtaacccggctccgccgagcggggcagcacctcacgcgctggagtcccgttgcgccctggtagaggcgccacgatggcaggggcgttgtcattttgatccactatgaggatgttgacagtggcgttaccagccagcgcctgggggctgccagcgtcccgggcttccacctgaaaactgaagtccttcagctgctcatagtcgaaggagcgcagggcgtacaagtagccgttctcagagttgatagaaacgtaggtgaagacgctcatgccctggatctggcactcgaggatagagtaggcaagctgggcgttggcgccctcatcccggtcggtggcgctcaccgcgtagatgtaggcgccaggcacgttgttttcagtcacatacacgtcgtagaccggctggctgaaacgcggcgcgttgtcgttcacatccgacacttgtacctggatcgacttactggtggagagcgcaggctcgccccggtcccgagccactacagtcagggtgtaggagtcccccgcctctcggtccaggggggcttcggtaacgatggtgtagtaattcttaaaggaagacttgaggcggaaaggcacgtctcccagtagctcgcactgcacctgcccattctcctctgagtcgcggtcagtcacgctgaaaagggccaccacagtgccgggcgccgcgccctcactcaccgcttccttcacggtgctgaagctgatctctggcgcgttgtcattagcatccagtactcgcactagcaccttgcagtgcgcaggcacggcgttggggcccaggtccttggcttgcacgtacacttggtacactgggctctcttcatagtccaactcgccgcttacctccagtctgccagtgcgcggcgagagtccgaaaagctcccgcgcccggggcgaaatgtggctgctgaaggagtacacgacctcaccgttctggccctcgtccgggtcggtggcgttgagctggatcacgagagtgcctgggggagagttctctggtagggacacagtgtagacgggttggtcgaaagcgggcacattgtcattggagtccagcactcggatggtgagtagggccgtgccggtgcgctgctgctgggggggcaggcctgctcccccgccacctccccctccttctcctactcctcccccacctcctccgtccaccgcggtcagcacgtagcggtgcaccgcttgctgctctcggtccagtggcttctccagcaccagctcagcgaatcggttgccatccccctgggtctgcacgtccagggagaagtagctgttgggggtgatctcgtagtcgcgcaaggagttggtgcccacgtctgggtcgaatgcgctctccaaggggaagcgagtgcctggcgtggcgctctcagagatttccaccgtcaggtctggctccgggaaagagggggggttgtcattaatgtccagcacctcgatctccacctggaacagctccagggggttctccagaaagacctccaggtgcaggacacaggaggggctctgtttgcagatttgttcgcggtctattttctcgttcacgtacagcacccctgtctccaggttgaggtctaagtaaggggtccttgagttgggcaccgtctgaaacccgcgagccgaaagttttgtaatgtccagacccagatcttcagcgatattccccacgaaagtgccatgttcctgctcctcctgtaccgtgtagtgaagctgggaaaagactccttccaccatccagagcaaggcaaacaataatagcacaatcatctccaaaaggaaaggaagtagcttcccgcagccagtcagccacccaatcacctcccccaccaccacgaaacaaaaaaaaatctgaaaaaatacaaataaaagtgcgctacgtgggggctcctgtggctttctgtctttaaaaatcttactccttttgcttcattttagagcttcccgcaatccagcctcatttttttttaaatcttagcacaggaagggtgacaggcgtcccctttcctcatctgtaatctttccactgactaattaataaaataacaataatacaatagtcagcgtcctttattccgacagtcttggcgctggcaaatcccaaagaggaaatttcgatatttcaagactgtcctcggtttgtcttcttgctgatgggaggagaacgaggaggaggaaaaagaggaggaggaggaggaagaagaagaagaggaagaggagaaggaaaaggagatgctgttggcaccgttaaacatgcctcttaatgtcaacggctggcaaatgcaaaagggcttaaaatcagcgatataattttgtgccggaaaagcacagaacggctctgcagcttaaaactttcattctcttcatttctccggatggatgttcttcttgacatttttttcctctttcgctctatttgtattttttgtctttcagagtcttggttccctctgtcctcatctccaccgttacttgcctctctgtaagtgtaatgagcagtttcttttctgctgttttcttcccaagcctctttccctctaacctgtctctttttccttccagtccttccttcctcctgcttcagcctctgagcctgtggtctgggctggcagtttct

SEQ ID NO: 16814 - RNA, 4846 nt, Homo sapiens
  source 1..4846: mol_type = other RNA
tacgtagatatatatgtattttaagcaagctatacctcttacataaattcagacagtagaaggagtgtgcaatcataatgcttattttatggaaacagtgaaaataattttaattatgacctaaatgcttttaagtaattaaagtcctcttgaattggatgtatagtataaagatattttccctaatttgcaaccatcctggtcaaaaagagctgaaaagttggtcagtaagtagaagtgccattaccaagtaagtttaaaacaaattcttcaaatttaaaaatgtaaaaattgtaaagtatcccaatccccccagctaatttagggaactgagcaagaagagaacattcttcagtttttaaatgacttttttttttttttttttggagatggggtcctgctctgtagcctaggctagagtgcagtggcatgatcagctcactgcaacctcaaactcctgggctcaagcaatcttcccacctcaacctcctgagtagctgggactacaggtgtgtgccaccatccccagctacttttataataaaatttctatgtagagacggagtcttcctacgttgcccaggctggtcttgaactcctgggctcaagcagtcttcctgcctcggcctcccaaagtgctggaattacaggcatgagccaccacactcagccttaaatgaagattttgtaaggaattgagcattcaactaaactcgtttttgtgagatggtcattttgttttaacctaacatggtttagagattattttatgaactctaagcattctggttcctcagttttctcaaagaaagagaactttagcaagtagcaggacaagctaccccacaccaatgccaccaggcgacaatactatgaataagtcaggaggcctcctagaatgcagccaaataggaaactgttccaaacagaatcagtcttgcatacttctgctcagaaggctcctctcgctttggaaactggaatgaggatcaccaacaggatcctcattttacacaggagttatgagagttacatcctctagcagagatgcttggtcattacctgtggtacatgagattaccgagctaaaagggaaaaaaaacgatcttaatgttctcccatgaactcaacttaagctttttatggaggcactgaggccatgcagctccttttccaaaagacacagataaaagccaaataaggtagaggactttggaaattttctctgaaaagttaaattccacataatagtaagactgtttgctgagagaaaactgacaagtaaaaactggtttaagagacagacattcaagacaaactgtattggaaatacaataatgaattttggcctgatagccctcatgctgtcttatagcaaaacactaaaattcatgcaacagagaaattggtgacatgaggactttttctccagacttcctggggaaaaactgtgagaatatacttttttcttctgtttgctttcgaaatgcattctttcttttgctgactttcccaaactttcccagtcgtttctgatgaaaaattcttcaataggaaaagaccaggtaaacttacatgaaagacatcaagtatcttttgagctccttctctctgccagaggagcaatcaactggattacacaaaactaccttcacaactaaaacaggtagaattggaacaggaattagttgtcattaatatactcgtaataaaataaagcttgttctgaaaccacaaggggtggtaagaagagactgtataaaagctactgggttctctagaaaatggatacagtatacagaatgtgagaagatacagaactcacactccagttataaaaatagacatggttctcagacaaaaagcaaatgagtacaaaagaattctccaaacgtgaactatttttaaaagatacatctatataaaacaacaagatgtcatctcagagctccaaagagtagtttgttgaaatggctgaaaaggggagatgaattggagacagataggtcaagaacccagaacagatgtgtcctactcttgtgtttggcagtgtacattggaggtcacaggcagatagactgcttttggtaatacatatataaataataatggctgactggttgatggtgcttgatggatgaatgagaaaacccaggttatcaaataatctcggtagttgaactgttagcttcttcacttgacaatgttgcacatcagaaatgattctaggttttttttacccagaatgatccctgccattcacaactcatgctccacgccccatggtttctattgtgccctaaaagatcagcctagactaatacataaatagaaaataactctggccttgaaatgaggggcagacaagtacttcatgctcagtacttataaatcacaaagaaatgctgaaattaatggtctgtctccttttactacaaaggagatgccatgagttaaagtcatgaaacaaagaaagtcaaaaagatatgggtagcagcacctttccatacccgcctggattttcaaggagcttttcactccttatgcctttcaaacaaaagttcatcagtttgaagaaaaagaaatggctctaaagttaaagagtccccagagaaaactaacagtacatgaaataggccctatgtgggcaaaaggacaagctgcagaaccagttaagacagaagaggcagcccaaggtcttactaaattacagttttagcatagtgtagcacaacatgggcagccctttttccatccaagcaacaattcagcaccatccacgtctggttcaaaagattactgaagtctgggctttcatctttggtaccacctcatgagttattcttggtttgcagtaggttcaaagaaacagaaaagctggtacctttgccttgtctgtgagtacaaacgctgggactctgattgctgcaaccattgaggccaattaaaataatactgtaacacacaggaatgatgcatccaattcctaatttccagataatagcagccatgcccctacagaggcgggatcatccatccccatcgtttaaggccttcggtttgttgtcctcagagtagaatagaacactgtgttcccacggacaaggaactccagatgaacccatggtctacatttggacagaattttaagtaccagatatgccaggcacagaaagaggactgacctgtggccatcatgcttggagaagcttctgttttggcacacaaactagaaacttcttagtgtattctggttttagttccctttcctgagtgaagcagccagggagtgaccaggttccataagccctcaatctgatacttggcattaattctctccatggtcttcttccacccaagctacaattttcccttcccatccagggatggcatcatcatcatggaaaatctcctctttgacagtgccaaactcaggatccagtgctttgaagtgataccggtgatttccttcccgatcaatagctgctttaaaatcctttaacgtcacctcctccaacctctttggtatattgaccatgaagggcgtaagtgaccggtcagtgaaatagagcactttagtacaggtgctgctgacagttggagagctctgtgagtgaggcaactttgagttagggggccaggactcccggtattcactacctacttgagttctgggtgacttgacccgaacctttctttcttgtttcttctgcgtctccataacatgcaggcgctccatgaggctagaaatgccctgctccaagctgtcaatagtgtggtgctgaggatcgtggccactgaagctgttgcgcaggctgcggagagcatctcgaacaagctgcaggtcgctggtccctctgttgctgactgaagtagctccttttcctgccgttggaaggagaaaaccattgctttgagagttgtgactgttgtagttggtcgcctcatctgcctctcttttcatacagtgagccaagaggacatctttgtgttctagctctcgctctagatccacctggtggtaactgacatcagagagtttccggagtgcttcttctaacttggcctggtgctgctgaagaaggcgatccttctgccccagctcttttttatattctcccaagagccggttcctctcatctagcttcctctgcagatccacattctggttgtgcagctcatctttgtccatatttgccctcagtagctcttgtttgagctgaagaacagatgtgtcctgctgagtcaatctctgctgcaaggcatcctttatcccctgtaagtttctggcttcttgtttacatttcagcagttccttctttaagtcctgattctcctccatactctgatccagacgactttggattataatcagttgttcctcgggattgacacctggttcacagagggccaagggcctctcctgttcatcttcaggtaaggatccattgagcagtaaggccctgggactagttcctttcgttaggtccatgctctggctctttcagctctctggacacctgactgctctgcttcaaggtgccttggccccagaagaaaatctgtagtcctgatatcattttctttgcttcctccatttctttttctaaatattcttgttgttccaacagctgttcttcccatgaggtctccagataggttccagggctccctggccgccagtctcgagataatggagaatctgtcccttctgttctgttctctattccttcagcgggaataatcacaaaatctgccttctcttctgactgggttataatggactcgctctttgcactgtggattggactgggtgaagtcaggcatttgacttgcgtccctccca

SEQ ID NO: 16815 - RNA, 5174 nt, Homo sapiens
  source 1..5174: mol_type = other RNA
tacgtagatatatatgtattttaagcaagctatacctcttacataaattcagacagtagaaggagtgtgcaatcataatgcttattttatggaaacagtgaaaataattttaattatgacctaaatgcttttaagtaattaaagtcctcttgaattggatgtatagtataaagatattttccctaatttgcaaccatcctggtcaaaaagagctgaaaagttggtcagtaagtagaagtgccattaccaagtaagtttaaaacaaattcttcaaatttaaaaatgtaaaaattgtaaagtatcccaatccccccagctaatttagggaactgagcaagaagagaacattcttcagtttttaaatgacttttttttttttttttttggagatggggtcctgctctgtagcctaggctagagtgcagtggcatgatcagctcactgcaacctcaaactcctgggctcaagcaatcttcccacctcaacctcctgagtagctgggactacaggtgtgtgccaccatccccagctacttttataataaaatttctatgtagagacggagtcttcctacgttgcccaggctggtcttgaactcctgggctcaagcagtcttcctgcctcggcctcccaaagtgctggaattacaggcatgagccaccacactcagccttaaatgaagattttgtaaggaattgagcattcaactaaactcgtttttgtgagatggtcattttgttttaacctaacatggtttagagattattttatgaactctaagcattctggttcctcagttttctcaaagaaagagaactttagcaagtagcaggacaagctaccccacaccaatgccaccaggcgacaatactatgaataagtcaggaggcctcctagaatgcagccaaataggaaactgttccaaacagaatcagtcttgcatacttctgctcagaaggctcctctcgctttggaaactggaatgaggatcaccaacaggatcctcattttacacaggagttatgagagttacatcctctagcagagatgcttggtcattacctgtggtacatgagattaccgagctaaaagggaaaaaaaacgatcttaatgttctcccatgaactcaacttaagctttttatggaggcactgaggccatgcagctccttttccaaaagacacagataaaagccaaataaggtagaggactttggaaattttctctgaaaagttaaattccacataatagtaagactgtttgctgagagaaaactgacaagtaaaaactggtttaagagacagacattcaagacaaactgtattggaaatacaataatgaattttggcctgatagccctcatgctgtcttatagcaaaacactaaaattcatgcaacagagaaattggtgacatgaggactttttctccagacttcctggggaaaaactgtgagaatatacttttttcttctgtttgctttcgaaatgcattctttcttttgctgactttcccaaactttcccagtcgtttctgatgaaaaattcttcaataggaaaagaccaggtaaacttacatgaaagacatcaagtatcttttgagctccttctctctgccagaggagcaatcaactggattacacaaaactaccttcacaactaaaacaggtagaattggaacaggaattagttgtcattaatatactcgtaataaaataaagcttgttctgaaaccacaaggggtggtaagaagagactgtataaaagctactgggttctctagaaaatggatacagtatacagaatgtgagaagatacagaactcacactccagttataaaaatagacatggttctcagacaaaaagcaaatgagtacaaaagaattctccaaacgtgaactatttttaaaagatacatctatataaaacaacaagatgtcatctcagagctccaaagagtagtttgttgaaatggctgaaaaggggagatgaattggagacagataggtcaagaacccagaacagatgtgtcctactcttgtgtttggcagtgtacattggaggtcacaggcagatagactgcttttggtaatacatatataaataataatggctgactggttgatggtgcttgatggatgaatgagaaaacccaggttatcaaataatctcggtagttgaactgttagcttcttcacttgacaatgttgcacatcagaaatgattctaggttttttttacccagaatgatccctgccattcacaactcatgctccacgccccatggtttctattgtgccctaaaagatcagcctagactaatacataaatagaaaataactctggccttgaaatgaggggcagacaagtacttcatgctcagtacttataaatcacaaagaaatgctgaaattaatggtctgtctccttttactacaaaggagatgccatgagttaaagtcatgaaacaaagaaagtcaaaaagatatgggtagcagcacctttccatacccgcctggattttcaaggagcttttcactccttatgcctttcaaacaaaagttcatcagtttgaagaaaaagaaatggctctaaagttaaagagtccccagagaaaactaacagtacatgaaataggccctatgtgggcaaaaggacaagctgcagaaccagttaagacagaagaggcagcccaaggtcttactaaattacagttttagcatagtgtagcacaacatgggcagccctttttccatccaagcaacaattcagcaccatccacgtctggttcaaaagattactgaagtctgggctttcatctttggtaccacctcatgagttattcttggtttgcagtaggttcaaagaaacagaaaagctggtacctttgccttgtctgtgagtacaaacgctgggactctgattgctgcaaccattgaggccaattaaaataatactgtaacacacaggaatgatgcatccaattcctaatttccagataatagcagccatgcccctacagaggcgggatcatccatccccatcgtttaaggccttcggtttgttgtcctcagagtagaatagaacactgtgttcccacggacaaggaactccagatgaacccatggtctacatttggacagaattttaagtaccagatatgccaggcacagaaagaggactgacctgtggccatcatgcttggagaagcttctgttttggcacacaaactagaaacttcttagtgtattctggttttagttccctttcctgagtgaagcagccagggagtgaccaggttccataagccctcaatctgatacttggcattaattctctccatggtcttcttccacccaagctacaattttcccttcccatccagggatggcatcatcatcatggaaaatctcctctttgacagtgccaaactcaggatccagtgctttgaagtgataccggtgatttccttcccgatcaatagctgctttaaaatcctttaacgtcacctcctccaacctctttggtatattgaccatgaagggcgtaagtgaccggtcagtgaaatagagcactttagtacaggtgctgctgacagttggagagctctgtgagtgaggcaactttgagttagggggccaggactcccggtattcactacctacttgagttctgggtgacttgacccgaacctttctttcttgtttcttctgcgtctccataacatgcaggcgctccatgaggctagaaatgccctgctccaagctgtcaatagtgtggtgctgaggatcgtggccactgaagctgttgcgcaggctgcggagagcatctcgaacaagctgcaggtcgctggtccctctgttgctgactgaagtagctccttttcctgccgttggaaggagaaaaccattgctttgagagttgtgactgttgtagttggtcgcctcatctgcctctcttttcatacagtgagccaagaggacatctttgtgttctagctctcgctctagatccacctggtggtaactgacatcagagagtttccggagtgcttcttctaacttggcctggtgctgctgaagaaggcgatccttctgccccagctcttttttatattctcccaagagccggttcctctcatctagcttcctctgcagatccacattctggttgtgcagctcatctttgtccatatttgccctcagtagctcttgtttgagctgaagaacagatgtgtcctgctgagtcaatctctgctgcaaggcatcctttatcccctgtaagtttctggcttcttgtttacatttcagcagttccttctttaagtcctgattctcctccatactctgatccagacgactttggattataatcagttgttcctcgggattgacacctggttcacagagggccaagggcctctcctgttcatcttcaggtaaggatccattgagcagtaaggcctgtagtcctgatatcattttctttgcttcctccatttctttttctaaatattcttgttgttccaacagctgttcttcccatgaggtctccagataggttccagggctccctggccgccagtctcgagataatggagaatctgtcccttctgttctgttctctattccttcagcgggaataatcacaaaatctgccttctcttctgactgggttataatggactcgctctttgcactgtggattggactgggtgaagtcaggcatttgacttgcgtccctcccatggtccccctcctgtctcgggcttcagcaagcctgcgtccccgggtgaagtgggaggctgagagtcacatcgctcccaaattcaggcatgtctccccgcgctggggctggaaaacgcctccacgggaaggccagctagcaaagctactggcccggctcgcgggagaaagcgggaacggcggcggcggcggcgtctcggccccagcgactgggatgctccaggctctgaagcgcgcagtcccggccgctcagactgtgcagcagcccggccccggcggaagctgcctcccctcgcaggctgccggcccctggccgctgcatcttggcctccgcggacgcacggtgccgggcatcccccctggcgggggcatctcaacccatctcccactgggagggaggctcccggcggcgcaggctgcgcctcgagtc

SEQ ID NO: 16816 - RNA, 5524 nt, Homo sapiens
  source 1..5524: mol_type = other RNA
tacgtagatatatatgtattttaagcaagctatacctcttacataaattcagacagtagaaggagtgtgcaatcataatgcttattttatggaaacagtgaaaataattttaattatgacctaaatgcttttaagtaattaaagtcctcttgaattggatgtatagtataaagatattttccctaatttgcaaccatcctggtcaaaaagagctgaaaagttggtcagtaagtagaagtgccattaccaagtaagtttaaaacaaattcttcaaatttaaaaatgtaaaaattgtaaagtatcccaatccccccagctaatttagggaactgagcaagaagagaacattcttcagtttttaaatgacttttttttttttttttttggagatggggtcctgctctgtagcctaggctagagtgcagtggcatgatcagctcactgcaacctcaaactcctgggctcaagcaatcttcccacctcaacctcctgagtagctgggactacaggtgtgtgccaccatccccagctacttttataataaaatttctatgtagagacggagtcttcctacgttgcccaggctggtcttgaactcctgggctcaagcagtcttcctgcctcggcctcccaaagtgctggaattacaggcatgagccaccacactcagccttaaatgaagattttgtaaggaattgagcattcaactaaactcgtttttgtgagatggtcattttgttttaacctaacatggtttagagattattttatgaactctaagcattctggttcctcagttttctcaaagaaagagaactttagcaagtagcaggacaagctaccccacaccaatgccaccaggcgacaatactatgaataagtcaggaggcctcctagaatgcagccaaataggaaactgttccaaacagaatcagtcttgcatacttctgctcagaaggctcctctcgctttggaaactggaatgaggatcaccaacaggatcctcattttacacaggagttatgagagttacatcctctagcagagatgcttggtcattacctgtggtacatgagattaccgagctaaaagggaaaaaaaacgatcttaatgttctcccatgaactcaacttaagctttttatggaggcactgaggccatgcagctccttttccaaaagacacagataaaagccaaataaggtagaggactttggaaattttctctgaaaagttaaattccacataatagtaagactgtttgctgagagaaaactgacaagtaaaaactggtttaagagacagacattcaagacaaactgtattggaaatacaataatgaattttggcctgatagccctcatgctgtcttatagcaaaacactaaaattcatgcaacagagaaattggtgacatgaggactttttctccagacttcctggggaaaaactgtgagaatatacttttttcttctgtttgctttcgaaatgcattctttcttttgctgactttcccaaactttcccagtcgtttctgatgaaaaattcttcaataggaaaagaccaggtaaacttacatgaaagacatcaagtatcttttgagctccttctctctgccagaggagcaatcaactggattacacaaaactaccttcacaactaaaacaggtagaattggaacaggaattagttgtcattaatatactcgtaataaaataaagcttgttctgaaaccacaaggggtggtaagaagagactgtataaaagctactgggttctctagaaaatggatacagtatacagaatgtgagaagatacagaactcacactccagttataaaaatagacatggttctcagacaaaaagcaaatgagtacaaaagaattctccaaacgtgaactatttttaaaagatacatctatataaaacaacaagatgtcatctcagagctccaaagagtagtttgttgaaatggctgaaaaggggagatgaattggagacagataggtcaagaacccagaacagatgtgtcctactcttgtgtttggcagtgtacattggaggtcacaggcagatagactgcttttggtaatacatatataaataataatggctgactggttgatggtgcttgatggatgaatgagaaaacccaggttatcaaataatctcggtagttgaactgttagcttcttcacttgacaatgttgcacatcagaaatgattctaggttttttttacccagaatgatccctgccattcacaactcatgctccacgccccatggtttctattgtgccctaaaagatcagcctagactaatacataaatagaaaataactctggccttgaaatgaggggcagacaagtacttcatgctcagtacttataaatcacaaagaaatgctgaaattaatggtctgtctccttttactacaaaggagatgccatgagttaaagtcatgaaacaaagaaagtcaaaaagatatgggtagcagcacctttccatacccgcctggattttcaaggagcttttcactccttatgcctttcaaacaaaagttcatcagtttgaagaaaaagaaatggctctaaagttaaagagtccccagagaaaactaacagtacatgaaataggccctatgtgggcaaaaggacaagctgcagaaccagttaagacagaagaggcagcccaaggtcttactaaattacagttttagcatagtgtagcacaacatgggcagccctttttccatccaagcaacaattcagcaccatccacgtctggttcaaaagattactgaagtctgggctttcatctttggtaccacctcatgagttattcttggtttgcagtaggttcaaagaaacagaaaagctggtacctttgccttgtctgtgagtacaaacgctgggactctgattgctgcaaccattgaggccaattaaaataatactgtaacacacaggaatgatgcatccaattcctaatttccagataatagcagccatgcccctacagaggcgggatcatccatccccatcgtttaaggccttcggtttgttgtcctcagagtagaatagaacactgtgttcccacggacaaggaactccagatgaacccatggtctacatttggacagaattttaagtaccagatatgccaggcacagaaagaggactgacctgtggccatcatgcttggagaagcttctgttttggcacacaaactagaaacttcttagtgtattctggttttagttccctttcctgagtgaagcagccagggagtgaccaggttccataagccctcaatctgatacttggcattaattctctccatggtcttcttccacccaagctacaattttcccttcccatccagggatggcatcatcatcatggaaaatctcctctttgacagtgccaaactcaggatccagtgctttgaagtgataccggtgatttccttcccgatcaatagctgctttaaaatcctttaacgtcacctcctccaacctctttggtatattgaccatgaagggcgtaagtgaccggtcagtgaaatagagcactttagtacaggtgctgctgacagttggagagctctgtgagtgaggcaactttgagttagggggccaggactcccggtattcactacctacttgagttctgggtgacttgacccgaacctttctttcttgtttcttctgcgtctccataacatgcaggcgctccatgaggctagaaatgccctgctccaagctgtcaatagtgtggtgctgaggatcgtggccactgaagctgttgcgcaggctgcggagagcatctcgaacaagctgcaggtcgctggtccctctgttgctgactgaagtagctccttttcctgccgttggaaggagaaaaccattgctttgagagttgtgactgttgtagttggtcgcctcatctgcctctcttttcatacagtgagccaagaggacatctttgtgttctagctctcgctctagatccacctggtggtaactgacatcagagagtttccggagtgcttcttctaacttggcctggtgctgctgaagaaggcgatccttctgccccagctcttttttatattctcccaagagccggttcctctcatctagcttcctctgcagatccacattctggttgtgcagctcatctttgtccatatttgccctcagtagctcttgtttgagctgaagaacagatgtgtcctgctgagtcaatctctgctgcaaggcatcctttatcccctgtaagtttctggcttcttgtttacatttcagcagttccttctttaagtcctgattctcctccatactctgatccagacgactttggattataatcagttgttcctcgggattgacacctggttcacagagggccaagggcctctcctgttcatcttcaggtaaggatccattgagcagtaaggcctgtagtcctgatatcattttctttgcttcctccatttctttttctaaatattcttgttgttccaacagctgttcttcccatgaggtctccagataggttccagggctccctggccgccagtctcgagataatggagaatctgtcccttctgttctgttctctattccttcagcgggaataatcacaaaatctgccttctcttctgactgggttataatggactcgctctttgcactgtggattggactgggtgaagtcaggctctgtctatatcgaaagacatcccgtcctgatcgggacatgtcatgacacacatcggccagagcagcagctgctccctgggcaacagcagtggcacagtgtggtcggtgactttgcagaggggctctggagtcccgtccttggttcaccgtcctgctggagccaggtttgaaatgagctgccaaggcaaggaccagcctcatgatagacttcaggtttccatccacaatatctttagccgaagtctggtgcatacgaatctttttagaggccacaaactgtagcactttctccacattattcttcatctcctgttggttaccgggactcagctgtaccccactcagcttttctcctgcaacaatctcgatgagatatgccaggatcaccccatcccggagatcttgtcgcaggtcctgcacaggcttcactgctggcctcttcttcagctgtgcattcacccaggccacataggcctgcagctgttgagaaggctctgttggcagcaaggagttattgaatctcataaccacttgggtccccatcttcaagagtccctagaagagacgaatcagggccatctcttaaatgatgggtccgtctggttcagcatctctgtccccagccctcctgagctcggcctgccagtgctctggctttgccgcggtttcccgctgccatggtgatgcgggggccggccacaagccccgcccgactccagccagccagagccagcccctgccggccttggtcccgcctctggcccgccggatcccgcctcctgcaggcccagaccgcgc

SEQ ID NO: 16817 - RNA, 5826 nt, Homo sapiens
  source 1..5826: mol_type = other RNA
tacgtagatatatatgtattttaagcaagctatacctcttacataaattcagacagtagaaggagtgtgcaatcataatgcttattttatggaaacagtgaaaataattttaattatgacctaaatgcttttaagtaattaaagtcctcttgaattggatgtatagtataaagatattttccctaatttgcaaccatcctggtcaaaaagagctgaaaagttggtcagtaagtagaagtgccattaccaagtaagtttaaaacaaattcttcaaatttaaaaatgtaaaaattgtaaagtatcccaatccccccagctaatttagggaactgagcaagaagagaacattcttcagtttttaaatgacttttttttttttttttttggagatggggtcctgctctgtagcctaggctagagtgcagtggcatgatcagctcactgcaacctcaaactcctgggctcaagcaatcttcccacctcaacctcctgagtagctgggactacaggtgtgtgccaccatccccagctacttttataataaaatttctatgtagagacggagtcttcctacgttgcccaggctggtcttgaactcctgggctcaagcagtcttcctgcctcggcctcccaaagtgctggaattacaggcatgagccaccacactcagccttaaatgaagattttgtaaggaattgagcattcaactaaactcgtttttgtgagatggtcattttgttttaacctaacatggtttagagattattttatgaactctaagcattctggttcctcagttttctcaaagaaagagaactttagcaagtagcaggacaagctaccccacaccaatgccaccaggcgacaatactatgaataagtcaggaggcctcctagaatgcagccaaataggaaactgttccaaacagaatcagtcttgcatacttctgctcagaaggctcctctcgctttggaaactggaatgaggatcaccaacaggatcctcattttacacaggagttatgagagttacatcctctagcagagatgcttggtcattacctgtggtacatgagattaccgagctaaaagggaaaaaaaacgatcttaatgttctcccatgaactcaacttaagctttttatggaggcactgaggccatgcagctccttttccaaaagacacagataaaagccaaataaggtagaggactttggaaattttctctgaaaagttaaattccacataatagtaagactgtttgctgagagaaaactgacaagtaaaaactggtttaagagacagacattcaagacaaactgtattggaaatacaataatgaattttggcctgatagccctcatgctgtcttatagcaaaacactaaaattcatgcaacagagaaattggtgacatgaggactttttctccagacttcctggggaaaaactgtgagaatatacttttttcttctgtttgctttcgaaatgcattctttcttttgctgactttcccaaactttcccagtcgtttctgatgaaaaattcttcaataggaaaagaccaggtaaacttacatgaaagacatcaagtatcttttgagctccttctctctgccagaggagcaatcaactggattacacaaaactaccttcacaactaaaacaggtagaattggaacaggaattagttgtcattaatatactcgtaataaaataaagcttgttctgaaaccacaaggggtggtaagaagagactgtataaaagctactgggttctctagaaaatggatacagtatacagaatgtgagaagatacagaactcacactccagttataaaaatagacatggttctcagacaaaaagcaaatgagtacaaaagaattctccaaacgtgaactatttttaaaagatacatctatataaaacaacaagatgtcatctcagagctccaaagagtagtttgttgaaatggctgaaaaggggagatgaattggagacagataggtcaagaacccagaacagatgtgtcctactcttgtgtttggcagtgtacattggaggtcacaggcagatagactgcttttggtaatacatatataaataataatggctgactggttgatggtgcttgatggatgaatgagaaaacccaggttatcaaataatctcggtagttgaactgttagcttcttcacttgacaatgttgcacatcagaaatgattctaggttttttttacccagaatgatccctgccattcacaactcatgctccacgccccatggtttctattgtgccctaaaagatcagcctagactaatacataaatagaaaataactctggccttgaaatgaggggcagacaagtacttcatgctcagtacttataaatcacaaagaaatgctgaaattaatggtctgtctccttttactacaaaggagatgccatgagttaaagtcatgaaacaaagaaagtcaaaaagatatgggtagcagcacctttccatacccgcctggattttcaaggagcttttcactccttatgcctttcaaacaaaagttcatcagtttgaagaaaaagaaatggctctaaagttaaagagtccccagagaaaactaacagtacatgaaataggccctatgtgggcaaaaggacaagctgcagaaccagttaagacagaagaggcagcccaaggtcttactaaattacagttttagcatagtgtagcacaacatgggcagccctttttccatccaagcaacaattcagcaccatccacgtctggttcaaaagattactgaagtctgggctttcatctttggtaccacctcatgagttattcttggtttgcagtaggttcaaagaaacagaaaagctggtacctttgccttgtctgtgagtacaaacgctgggactctgattgctgcaaccattgaggccaattaaaataatactgtaacacacaggaatgatgcatccaattcctaatttccagataatagcagccatgcccctacagaggcgggatcatccatccccatcgtttaaggccttcggtttgttgtcctcagagtagaatagaacactgtgttcccacggacaaggaactccagatgaacccatggtctacatttggacagaattttaagtaccagatatgccaggcacagaaagaggactgacctgtggccatcatgcttggagaagcttctgttttggcacacaaactagaaacttcttagtgtattctggttttagttccctttcctgagtgaagcagccagggagtgaccaggttccataagccctcaatctgatacttggcattaattctctccatggtcttcttccacccaagctacaattttcccttcccatccagggatggcatcatcatcatggaaaatctcctctttgacagtgccaaactcaggatccagtgctttgaagtgataccggtgatttccttcccgatcaatagctgctttaaaatcctttaacgtcacctcctccaacctctttggtatattgaccatgaagggcgtaagtgaccggtcagtgaaatagagcactttagtacaggtgctgctgacagttggagagctctgtgagtgaggcaactttgagttagggggccaggactcccggtattcactacctacttgagttctgggtgacttgacccgaacctttctttcttgtttcttctgcgtctccataacatgcaggcgctccatgaggctagaaatgccctgctccaagctgtcaatagtgtggtgctgaggatcgtggccactgaagctgttgcgcaggctgcggagagcatctcgaacaagctgcaggtcgctggtccctctgttgctgactgaagtagctccttttcctgccgttggaaggagaaaaccattgctttgagagttgtgactgttgtagttggtcgcctcatctgcctctcttttcatacagtgagccaagaggacatctttgtgttctagctctcgctctagatccacctggtggtaactgacatcagagagtttccggagtgcttcttctaacttggcctggtgctgctgaagaaggcgatccttctgccccagctcttttttatattctcccaagagccggttcctctcatctagcttcctctgcagatccacattctggttgtgcagctcatctttgtccatatttgccctcagtagctcttgtttgagctgaagaacagatgtgtcctgctgagtcaatctctgctgcaaggcatcctttatcccctgtaagtttctggcttcttgtttacatttcagcagttccttctttaagtcctgattctcctccatactctgatccagacgactttggattataatcagttgttcctcgggattgacacctggttcacagagggccaagggcctctcctgttcatcttcaggtaaggatccattgagcagtaaggcctgtagtcctgatatcattttctttgcttcctccatttctttttctaaatattcttgttgttccaacagctgttcttcccatgaggtctccagataggttccagggctccctggccgccagtctcgagataatggagaatctgtcccttctgttctgttctctattccttcagcgggaataatcacaaaatctgccttctcttctgactgggttataatggactcgctctttgcactgtggattggactgggtgaagtcaggctctgtctatatcgaaagacatcccgtcctgatcgggacatgtcatgacacacatcggccagagcagcagctgctccctgggcaacagcagtggcacagtgtggtcggtgactttgcagaggggctctggagtcccgtccttggttcaccgtcctgctggagccaggtttgaaatgagctgccaaggcaaggaccagcctcatgatagacttcaggtttccatccacaatatctttagccgaagtctggtgcatacgaatctttttagaggccacaaactgtagcactttctccacattattcttcatctcctgttggttaccgggactcagctgtaccccactcagcttttctcctgcaacaatctcgatgagatatgccaggatcaccccatcccggagatcttgtcgcaggtcctgcacaggcttcactgctggcctcttcttcagctgtgcattcacccaggccacataggcctgcagctgttgctcattgaagccctcctgcaggacgtccagtaagttccctcgggtcaggcaggctagcattgttcctgctgggggctccccgggcggggtctccagcccggcggccgccgccgcctcctcctcctccctctgcacacaaaggctctcggctcagctcattgggatccctccggagtcccgcatgccacttactggaaacctagactggagccaaactagcggcttgcactgggcatgctcgcacgggggcctccgctggaggggcccggcgcggtcgcggttcctatggaaacaactgggcgcgcactaggttgagcggcgctgccgggctgcccccagccccgctttcctgcgggaaagccgcacggccaggcgggctggcgagggcgcgcgctgcacgcccgcacgcacgcgcacaccccccccccgcccgggccgcagcacgggcgtgtgtgcgtgcgctacacacacacacactcacacggcttttaggcaaacgtgctgctgtatgtgcgcgctgtgtgcatacacacacacacacacatacacacatacacacatacacacacacacgttgacaaacaggcggcccggctggcgtatgcatgcgcttg

SEQ ID NO: 16818 - RNA, 5632 nt, Homo sapiens
  source 1..5632: mol_type = other RNA
tacgtagatatatatgtattttaagcaagctatacctcttacataaattcagacagtagaaggagtgtgcaatcataatgcttattttatggaaacagtgaaaataattttaattatgacctaaatgcttttaagtaattaaagtcctcttgaattggatgtatagtataaagatattttccctaatttgcaaccatcctggtcaaaaagagctgaaaagttggtcagtaagtagaagtgccattaccaagtaagtttaaaacaaattcttcaaatttaaaaatgtaaaaattgtaaagtatcccaatccccccagctaatttagggaactgagcaagaagagaacattcttcagtttttaaatgacttttttttttttttttttggagatggggtcctgctctgtagcctaggctagagtgcagtggcatgatcagctcactgcaacctcaaactcctgggctcaagcaatcttcccacctcaacctcctgagtagctgggactacaggtgtgtgccaccatccccagctacttttataataaaatttctatgtagagacggagtcttcctacgttgcccaggctggtcttgaactcctgggctcaagcagtcttcctgcctcggcctcccaaagtgctggaattacaggcatgagccaccacactcagccttaaatgaagattttgtaaggaattgagcattcaactaaactcgtttttgtgagatggtcattttgttttaacctaacatggtttagagattattttatgaactctaagcattctggttcctcagttttctcaaagaaagagaactttagcaagtagcaggacaagctaccccacaccaatgccaccaggcgacaatactatgaataagtcaggaggcctcctagaatgcagccaaataggaaactgttccaaacagaatcagtcttgcatacttctgctcagaaggctcctctcgctttggaaactggaatgaggatcaccaacaggatcctcattttacacaggagttatgagagttacatcctctagcagagatgcttggtcattacctgtggtacatgagattaccgagctaaaagggaaaaaaaacgatcttaatgttctcccatgaactcaacttaagctttttatggaggcactgaggccatgcagctccttttccaaaagacacagataaaagccaaataaggtagaggactttggaaattttctctgaaaagttaaattccacataatagtaagactgtttgctgagagaaaactgacaagtaaaaactggtttaagagacagacattcaagacaaactgtattggaaatacaataatgaattttggcctgatagccctcatgctgtcttatagcaaaacactaaaattcatgcaacagagaaattggtgacatgaggactttttctccagacttcctggggaaaaactgtgagaatatacttttttcttctgtttgctttcgaaatgcattctttcttttgctgactttcccaaactttcccagtcgtttctgatgaaaaattcttcaataggaaaagaccaggtaaacttacatgaaagacatcaagtatcttttgagctccttctctctgccagaggagcaatcaactggattacacaaaactaccttcacaactaaaacaggtagaattggaacaggaattagttgtcattaatatactcgtaataaaataaagcttgttctgaaaccacaaggggtggtaagaagagactgtataaaagctactgggttctctagaaaatggatacagtatacagaatgtgagaagatacagaactcacactccagttataaaaatagacatggttctcagacaaaaagcaaatgagtacaaaagaattctccaaacgtgaactatttttaaaagatacatctatataaaacaacaagatgtcatctcagagctccaaagagtagtttgttgaaatggctgaaaaggggagatgaattggagacagataggtcaagaacccagaacagatgtgtcctactcttgtgtttggcagtgtacattggaggtcacaggcagatagactgcttttggtaatacatatataaataataatggctgactggttgatggtgcttgatggatgaatgagaaaacccaggttatcaaataatctcggtagttgaactgttagcttcttcacttgacaatgttgcacatcagaaatgattctaggttttttttacccagaatgatccctgccattcacaactcatgctccacgccccatggtttctattgtgccctaaaagatcagcctagactaatacataaatagaaaataactctggccttgaaatgaggggcagacaagtacttcatgctcagtacttataaatcacaaagaaatgctgaaattaatggtctgtctccttttactacaaaggagatgccatgagttaaagtcatgaaacaaagaaagtcaaaaagatatgggtagcagcacctttccatacccgcctggattttcaaggagcttttcactccttatgcctttcaaacaaaagttcatcagtttgaagaaaaagaaatggctctaaagttaaagagtccccagagaaaactaacagtacatgaaataggccctatgtgggcaaaaggacaagctgcagaaccagttaagacagaagaggcagcccaaggtcttactaaattacagttttagcatagtgtagcacaacatgggcagccctttttccatccaagcaacaattcagcaccatccacgtctggttcaaaagattactgaagtctgggctttcatctttggtaccacctcatgagttattcttggtttgcagtaggttcaaagaaacagaaaagctggtacctttgccttgtctgtgagtacaaacgctgggactctgattgctgcaaccattgaggccaattaaaataatactgtaacacacaggaatgatgcatccaattcctaatttccagataatagcagccatgcccctacagaggcgggatcatccatccccatcgtttaaggccttcggtttgttgtcctcagagtagaatagaacactgtgttcccacggacaaggaactccagatgaacccatggtctacatttggacagaattttaagtaccagatatgccaggcacagaaagaggactgacctgtggccatcatgcttggagaagcttctgttttggcacacaaactagaaacttcttagtgtattctggttttagttccctttcctgagtgaagcagccagggagtgaccaggttccataagccctcaatctgatacttggcattaattctctccatggtcttcttccacccaagctacaattttcccttcccatccagggatggcatcatcatcatggaaaatctcctctttgacagtgccaaactcaggatccagtgctttgaagtgataccggtgatttccttcccgatcaatagctgctttaaaatcctttaacgtcacctcctccaacctctttggtatattgaccatgaagggcgtaagtgaccggtcagtgaaatagagcactttagtacaggtgctgctgacagttggagagctctgtgagtgaggcaactttgagttagggggccaggactcccggtattcactacctacttgagttctgggtgacttgacccgaacctttctttcttgtttcttctgcgtctccataacatgcaggcgctccatgaggctagaaatgccctgctccaagctgtcaatagtgtggtgctgaggatcgtggccactgaagctgttgcgcaggctgcggagagcatctcgaacaagctgcaggtcgctggtccctctgttgctgactgaagtagctccttttcctgccgttggaaggagaaaaccattgctttgagagttgtgactgttgtagttggtcgcctcatctgcctctcttttcatacagtgagccaagaggacatctttgtgttctagctctcgctctagatccacctggtggtaactgacatcagagagtttccggagtgcttcttctaacttggcctggtgctgctgaagaaggcgatccttctgccccagctcttttttatattctcccaagagccggttcctctcatctagcttcctctgcagatccacattctggttgtgcagctcatctttgtccatatttgccctcagtagctcttgtttgagctgaagaacagatgtgtcctgctgagtcaatctctgctgcaaggcatcctttatcccctgtaagtttctggcttcttgtttacatttcagcagttccttctttaagtcctgattctcctccatactctgatccagacgactttggattataatcagttgttcctcgggattgacacctggttcacagagggccaagggcctctcctgttcatcttcaggtaaggatccattgagcagtaaggcctgtagtcctgatatcattttctttgcttcctccatttctttttctaaatattcttgttgttccaacagctgttcttcccatgaggtctccagataggttccagggctccctggccgccagtctcgagataatggagaatctgtcccttctgttctgttctctattccttcagcgggaataatcacaaaatctgccttctcttctgactgggttataatggactcgctctttgcactgtggattggactgggtgaagtcaggctggagcagctggattcagacggggacctttgttgcccttcgtactgctgcactagggcccgcacactccagtatggattctcaatttcctcatccatgctgctgttcctctgtctatatcgaaagacatcccgtcctgatcgggacatgtcatgacacacatcggccagagcagcagctgctccctgggcaacagcagtggcacagtgtggtcggtgactttgcagaggggctctggagtcccgtccttggttcaccgtcctgctggagccaggtttgaaatgagctgccaaggcaaggaccagcctcatgatagacttcaggtttccatccacaatatctttagccgaagtctggtgcatacgaatctttttagaggccacaaactgtagcactttctccacattattcttcatctcctgttggttaccgggactcagctgtaccccactcagcttttctcctgcaacaatctcgatgagatatgccaggatcaccccatcccggagatcttgtcgcaggtcctgcacaggcttcactgctggcctcttcttcagctgtgcattcacccaggccacataggcctgcagctgttgagaaggctctgttggcagcaaggagttattgaatctcataaccacttgggtccccatcttcaagagtccctagaagagacgaatcagggccatctcttaaatgatgggtccgtctggttcagcatctctgtccccagccctcctgagctcggcctgccagtgctctggctttgccgcggtttcccgctgccatggtgatgcgggggccggccacaagccccgcccgactccagccagccagagccagcccctgccggccttggtcccgcctctggcccgccggatcccgcctcctgcaggcccagaccgcgc

SEQ ID NO: 16819 - RNA, 5505 nt, Homo sapiens
  source 1..5505: mol_type = other RNA
tacgtagatatatatgtattttaagcaagctatacctcttacataaattcagacagtagaaggagtgtgcaatcataatgcttattttatggaaacagtgaaaataattttaattatgacctaaatgcttttaagtaattaaagtcctcttgaattggatgtatagtataaagatattttccctaatttgcaaccatcctggtcaaaaagagctgaaaagttggtcagtaagtagaagtgccattaccaagtaagtttaaaacaaattcttcaaatttaaaaatgtaaaaattgtaaagtatcccaatccccccagctaatttagggaactgagcaagaagagaacattcttcagtttttaaatgacttttttttttttttttttggagatggggtcctgctctgtagcctaggctagagtgcagtggcatgatcagctcactgcaacctcaaactcctgggctcaagcaatcttcccacctcaacctcctgagtagctgggactacaggtgtgtgccaccatccccagctacttttataataaaatttctatgtagagacggagtcttcctacgttgcccaggctggtcttgaactcctgggctcaagcagtcttcctgcctcggcctcccaaagtgctggaattacaggcatgagccaccacactcagccttaaatgaagattttgtaaggaattgagcattcaactaaactcgtttttgtgagatggtcattttgttttaacctaacatggtttagagattattttatgaactctaagcattctggttcctcagttttctcaaagaaagagaactttagcaagtagcaggacaagctaccccacaccaatgccaccaggcgacaatactatgaataagtcaggaggcctcctagaatgcagccaaataggaaactgttccaaacagaatcagtcttgcatacttctgctcagaaggctcctctcgctttggaaactggaatgaggatcaccaacaggatcctcattttacacaggagttatgagagttacatcctctagcagagatgcttggtcattacctgtggtacatgagattaccgagctaaaagggaaaaaaaacgatcttaatgttctcccatgaactcaacttaagctttttatggaggcactgaggccatgcagctccttttccaaaagacacagataaaagccaaataaggtagaggactttggaaattttctctgaaaagttaaattccacataatagtaagactgtttgctgagagaaaactgacaagtaaaaactggtttaagagacagacattcaagacaaactgtattggaaatacaataatgaattttggcctgatagccctcatgctgtcttatagcaaaacactaaaattcatgcaacagagaaattggtgacatgaggactttttctccagacttcctggggaaaaactgtgagaatatacttttttcttctgtttgctttcgaaatgcattctttcttttgctgactttcccaaactttcccagtcgtttctgatgaaaaattcttcaataggaaaagaccaggtaaacttacatgaaagacatcaagtatcttttgagctccttctctctgccagaggagcaatcaactggattacacaaaactaccttcacaactaaaacaggtagaattggaacaggaattagttgtcattaatatactcgtaataaaataaagcttgttctgaaaccacaaggggtggtaagaagagactgtataaaagctactgggttctctagaaaatggatacagtatacagaatgtgagaagatacagaactcacactccagttataaaaatagacatggttctcagacaaaaagcaaatgagtacaaaagaattctccaaacgtgaactatttttaaaagatacatctatataaaacaacaagatgtcatctcagagctccaaagagtagtttgttgaaatggctgaaaaggggagatgaattggagacagataggtcaagaacccagaacagatgtgtcctactcttgtgtttggcagtgtacattggaggtcacaggcagatagactgcttttggtaatacatatataaataataatggctgactggttgatggtgcttgatggatgaatgagaaaacccaggttatcaaataatctcggtagttgaactgttagcttcttcacttgacaatgttgcacatcagaaatgattctaggttttttttacccagaatgatccctgccattcacaactcatgctccacgccccatggtttctattgtgccctaaaagatcagcctagactaatacataaatagaaaataactctggccttgaaatgaggggcagacaagtacttcatgctcagtacttataaatcacaaagaaatgctgaaattaatggtctgtctccttttactacaaaggagatgccatgagttaaagtcatgaaacaaagaaagtcaaaaagatatgggtagcagcacctttccatacccgcctggattttcaaggagcttttcactccttatgcctttcaaacaaaagttcatcagtttgaagaaaaagaaatggctctaaagttaaagagtccccagagaaaactaacagtacatgaaataggccctatgtgggcaaaaggacaagctgcagaaccagttaagacagaagaggcagcccaaggtcttactaaattacagttttagcatagtgtagcacaacatgggcagccctttttccatccaagcaacaattcagcaccatccacgtctggttcaaaagattactgaagtctgggctttcatctttggtaccacctcatgagttattcttggtttgcagtaggttcaaagaaacagaaaagctggtacctttgccttgtctgtgagtacaaacgctgggactctgattgctgcaaccattgaggccaattaaaataatactgtaacacacaggaatgatgcatccaattcctaatttccagataatagcagccatgcccctacagaggcgggatcatccatccccatcgtttaaggccttcggtttgttgtcctcagagtagaatagaacactgtgttcccacggacaaggaactccagatgaacccatggtctacatttggacagaattttaagtaccagatatgccaggcacagaaagaggactgacctgtggccatcatgcttggagaagcttctgttttggcacacaaactagaaacttcttagtgtattctggttttagttccctttcctgagtgaagcagccagggagtgaccaggttccataagccctcaatctgatacttggcattaattctctccatggtcttcttccacccaagctacaattttcccttcccatccagggatggcatcatcatcatggaaaatctcctctttgacagtgccaaactcaggatccagtgctttgaagtgataccggtgatttccttcccgatcaatagctgctttaaaatcctttaacgtcacctcctccaacctctttggtatattgaccatgaagggcgtaagtgaccggtcagtgaaatagagcactttagtacaggtgctgctgacagttggagagctctgtgagtgaggcaactttgagttagggggccaggactcccggtattcactacctacttgagttctgggtgacttgacccgaacctttctttcttgtttcttctgcgtctccataacatgcaggcgctccatgaggctagaaatgccctgctccaagctgtcaatagtgtggtgctgaggatcgtggccactgaagctgttgcgcaggctgcggagagcatctcgaacaagctgcaggtcgctggtccctctgttgctgactgaagtagctccttttcctgccgttggaaggagaaaaccattgctttgagagttgtgactgttgtagttggtcgcctcatctgcctctcttttcatacagtgagccaagaggacatctttgtgttctagctctcgctctagatccacctggtggtaactgacatcagagagtttccggagtgcttcttctaacttggcctggtgctgctgaagaaggcgatccttctgccccagctcttttttatattctcccaagagccggttcctctcatctagcttcctctgcagatccacattctggttgtgcagctcatctttgtccatatttgccctcagtagctcttgtttgagctgaagaacagatgtgtcctgctgagtcaatctctgctgcaaggcatcctttatcccctgtaagtttctggcttcttgtttacatttcagcagttccttctttaagtcctgattctcctccatactctgatccagacgactttggattataatcagttgttcctcgggattgacacctggttcacagagggccaagggcctctcctgttcatcttcaggtaaggatccattgagcagtaaggcctgtagtcctgatatcattttctttgcttcctccatttctttttctaaatattcttgttgttccaacagctgttcttcccatgaggtctccagataggttccagggctccctggccgccagtctcgagataatggagaatctgtcccttctgttctgttctctattccttcagcgggaataatcacaaaatctgccttctcttctgactgggttataatggactcgctctttgcactgtggattggactgggtgaagtcaggctggagcagctggattcagacggggacctttgttgcccttcgtactgctgcactagggcccgcacactccagtatggattctcaatttcctcatccatgctgctgttcctctgtctatatcgaaagacatcccgtcctgatcgggacatgtcatgacacacatcggccagagcagcagctgctccctgggcaacagcagtggcacagtgtggtcggtgactttgcagaggggctctggagtcccgtccttggttcaccgtcctgctggagccaggtttgaaatgagctgccaaggcaaggaccagcctcatgatagacttcaggtttccatccacaatatctttagccgaagtctggtgcatacgaatctttttagaggccacaaactgtagcactttctccacattattcttcatctcctgttggttaccgggactcagctgtaccccactcagcttttctcctgcaacaatctcgatgagatatgccaggatcaccccatcccggagatcttgtcgcaggtcctgcacaggcttcactgctggcctcttcttcagctgtgcattcacccaggccacataggcctgcagctgttgagaaggctctgttggcagcaaggagttattgaatctcataaccacttgggtccccatcttcaagagtccctcttaaatgatgggtccgtctggttcagcatctctgtccccagccctcctgagctcggcctgccagtgctctggctttgccgcggtttcccgctgccatggtgatgcgggggccg

SEQ ID NO: 16820 - RNA, 5537 nt, Homo sapiens
  source 1..5537: mol_type = other RNA
tacgtagatatatatgtattttaagcaagctatacctcttacataaattcagacagtagaaggagtgtgcaatcataatgcttattttatggaaacagtgaaaataattttaattatgacctaaatgcttttaagtaattaaagtcctcttgaattggatgtatagtataaagatattttccctaatttgcaaccatcctggtcaaaaagagctgaaaagttggtcagtaagtagaagtgccattaccaagtaagtttaaaacaaattcttcaaatttaaaaatgtaaaaattgtaaagtatcccaatccccccagctaatttagggaactgagcaagaagagaacattcttcagtttttaaatgacttttttttttttttttttggagatggggtcctgctctgtagcctaggctagagtgcagtggcatgatcagctcactgcaacctcaaactcctgggctcaagcaatcttcccacctcaacctcctgagtagctgggactacaggtgtgtgccaccatccccagctacttttataataaaatttctatgtagagacggagtcttcctacgttgcccaggctggtcttgaactcctgggctcaagcagtcttcctgcctcggcctcccaaagtgctggaattacaggcatgagccaccacactcagccttaaatgaagattttgtaaggaattgagcattcaactaaactcgtttttgtgagatggtcattttgttttaacctaacatggtttagagattattttatgaactctaagcattctggttcctcagttttctcaaagaaagagaactttagcaagtagcaggacaagctaccccacaccaatgccaccaggcgacaatactatgaataagtcaggaggcctcctagaatgcagccaaataggaaactgttccaaacagaatcagtcttgcatacttctgctcagaaggctcctctcgctttggaaactggaatgaggatcaccaacaggatcctcattttacacaggagttatgagagttacatcctctagcagagatgcttggtcattacctgtggtacatgagattaccgagctaaaagggaaaaaaaacgatcttaatgttctcccatgaactcaacttaagctttttatggaggcactgaggccatgcagctccttttccaaaagacacagataaaagccaaataaggtagaggactttggaaattttctctgaaaagttaaattccacataatagtaagactgtttgctgagagaaaactgacaagtaaaaactggtttaagagacagacattcaagacaaactgtattggaaatacaataatgaattttggcctgatagccctcatgctgtcttatagcaaaacactaaaattcatgcaacagagaaattggtgacatgaggactttttctccagacttcctggggaaaaactgtgagaatatacttttttcttctgtttgctttcgaaatgcattctttcttttgctgactttcccaaactttcccagtcgtttctgatgaaaaattcttcaataggaaaagaccaggtaaacttacatgaaagacatcaagtatcttttgagctccttctctctgccagaggagcaatcaactggattacacaaaactaccttcacaactaaaacaggtagaattggaacaggaattagttgtcattaatatactcgtaataaaataaagcttgttctgaaaccacaaggggtggtaagaagagactgtataaaagctactgggttctctagaaaatggatacagtatacagaatgtgagaagatacagaactcacactccagttataaaaatagacatggttctcagacaaaaagcaaatgagtacaaaagaattctccaaacgtgaactatttttaaaagatacatctatataaaacaacaagatgtcatctcagagctccaaagagtagtttgttgaaatggctgaaaaggggagatgaattggagacagataggtcaagaacccagaacagatgtgtcctactcttgtgtttggcagtgtacattggaggtcacaggcagatagactgcttttggtaatacatatataaataataatggctgactggttgatggtgcttgatggatgaatgagaaaacccaggttatcaaataatctcggtagttgaactgttagcttcttcacttgacaatgttgcacatcagaaatgattctaggttttttttacccagaatgatccctgccattcacaactcatgctccacgccccatggtttctattgtgccctaaaagatcagcctagactaatacataaatagaaaataactctggccttgaaatgaggggcagacaagtacttcatgctcagtacttataaatcacaaagaaatgctgaaattaatggtctgtctccttttactacaaaggagatgccatgagttaaagtcatgaaacaaagaaagtcaaaaagatatgggtagcagcacctttccatacccgcctggattttcaaggagcttttcactccttatgcctttcaaacaaaagttcatcagtttgaagaaaaagaaatggctctaaagttaaagagtccccagagaaaactaacagtacatgaaataggccctatgtgggcaaaaggacaagctgcagaaccagttaagacagaagaggcagcccaaggtcttactaaattacagttttagcatagtgtagcacaacatgggcagccctttttccatccaagcaacaattcagcaccatccacgtctggttcaaaagattactgaagtctgggctttcatctttggtaccacctcatgagttattcttggtttgcagtaggttcaaagaaacagaaaagctggtacctttgccttgtctgtgagtacaaacgctgggactctgattgctgcaaccattgaggccaattaaaataatactgtaacacacaggaatgatgcatccaattcctaatttccagataatagcagccatgcccctacagaggcgggatcatccatccccatcgtttaaggccttcggtttgttgtcctcagagtagaatagaacactgtgttcccacggacaaggaactccagatgaacccatggtctacatttggacagaattttaagtaccagatatgccaggcacagaaagaggactgacctgtggccatcatgcttggagaagcttctgttttggcacacaaactagaaacttcttagtgtattctggttttagttccctttcctgagtgaagcagccagggagtgaccaggttccataagccctcaatctgatacttggcattaattctctccatggtcttcttccacccaagctacaattttcccttcccatccagggatggcatcatcatcatggaaaatctcctctttgacagtgccaaactcaggatccagtgctttgaagtgataccggtgatttccttcccgatcaatagctgctttaaaatcctttaacgtcacctcctccaacctctttggtatattgaccatgaagggcgtaagtgaccggtcagtgaaatagagcactttagtacaggtgctgctgacagttggagagctctgtgagtgaggcaactttgagttagggggccaggactcccggtattcactacctacttgagttctgggtgacttgacccgaacctttctttcttgtttcttctgcgtctccataacatgcaggcgctccatgaggctagaaatgccctgctccaagctgtcaatagtgtggtgctgaggatcgtggccactgaagctgttgcgcaggctgcggagagcatctcgaacaagctgcaggtcgctggtccctctgttgctgactgaagtagctccttttcctgccgttggaaggagaaaaccattgctttgagagttgtgactgttgtagttggtcgcctcatctgcctctcttttcatacagtgagccaagaggacatctttgtgttctagctctcgctctagatccacctggtggtaactgacatcagagagtttccggagtgcttcttctaacttggcctggtgctgctgaagaaggcgatccttctgccccagctcttttttatattctcccaagagccggttcctctcatctagcttcctctgcagatccacattctggttgtgcagctcatctttgtccatatttgccctcagtagctcttgtttgagctgaagaacagatgtgtcctgctgagtcaatctctgctgcaaggcatcctttatcccctgtaagtttctggcttcttgtttacatttcagcagttccttctttaagtcctgattctcctccatactctgatccagacgactttggattataatcagttgttcctcgggattgacacctggttcacagagggccaagggcctctcctgttcatcttcaggtaaggatccattgagcagtaaggcctgtagtcctgatatcattttctttgcttcctccatttctttttctaaatattcttgttgttccaacagctgttcttcccatgaggtctccagataggttccagggctccctggccgccagtctcgagataatggagaatctgtcccttctgttctgttctctattccttcagcgggaataatcacaaaatctgccttctcttctgactgggttataatggactcgctctttgcactgtggattggactgggtgaagtcaggctggagcagctggattcagacggggacctttgttgcccttcgtactgctgcactagggcccgcacactccagtatggattctcaatttcctcatccatgctgctgttcctctgtctatatcgaaagacatcccgtcctgatcgggacatgtcatgacacacatcggccagagcagcagctgctccctgggcaacagcagtggcacagtgtggtcggtgactttgcagaggggctctggagtcccgtccttggttcaccgtcctgctggagccaggtttgaaatgagctgccaaggcaaggaccagcctcatgatagacttcaggtttccatccacaatatctttagccgaagtctggtgcatacgaatctttttagaggccacaaactgtagcactttctccacattattcttcatctcctgttggttaccgggactcagctgtaccccactcagcttttctcctgcaacaatctcgatgagatatgccaggatcaccccatcccggagatcttgtcgcaggtcctgcacaggcttcactgctggcctcttcttcagctgtgcattcacccaggccacataggcctgcagctgttgctcattgaagccctcctgcaggacgtccagtaagttccctcgggtcaggcaggctagcattgttcctgctgggggctccccgggcggggtctccagcccggcggccgccgccgcctcctcctcctccctctgcacacaaaggctctcggctcagctcattgggatccctccggagtcccgcatgccacttactggaaacctagactggagccaaact

SEQ ID NO: 16821 - RNA, 4821 nt, Homo sapiens
  source 1..4821: mol_type = other RNA
tacgtagatatatatgtattttaagcaagctatacctcttacataaattcagacagtagaaggagtgtgcaatcataatgcttattttatggaaacagtgaaaataattttaattatgacctaaatgcttttaagtaattaaagtcctcttgaattggatgtatagtataaagatattttccctaatttgcaaccatcctggtcaaaaagagctgaaaagttggtcagtaagtagaagtgccattaccaagtaagtttaaaacaaattcttcaaatttaaaaatgtaaaaattgtaaagtatcccaatccccccagctaatttagggaactgagcaagaagagaacattcttcagtttttaaatgacttttttttttttttttttggagatggggtcctgctctgtagcctaggctagagtgcagtggcatgatcagctcactgcaacctcaaactcctgggctcaagcaatcttcccacctcaacctcctgagtagctgggactacaggtgtgtgccaccatccccagctacttttataataaaatttctatgtagagacggagtcttcctacgttgcccaggctggtcttgaactcctgggctcaagcagtcttcctgcctcggcctcccaaagtgctggaattacaggcatgagccaccacactcagccttaaatgaagattttgtaaggaattgagcattcaactaaactcgtttttgtgagatggtcattttgttttaacctaacatggtttagagattattttatgaactctaagcattctggttcctcagttttctcaaagaaagagaactttagcaagtagcaggacaagctaccccacaccaatgccaccaggcgacaatactatgaataagtcaggaggcctcctagaatgcagccaaataggaaactgttccaaacagaatcagtcttgcatacttctgctcagaaggctcctctcgctttggaaactggaatgaggatcaccaacaggatcctcattttacacaggagttatgagagttacatcctctagcagagatgcttggtcattacctgtggtacatgagattaccgagctaaaagggaaaaaaaacgatcttaatgttctcccatgaactcaacttaagctttttatggaggcactgaggccatgcagctccttttccaaaagacacagataaaagccaaataaggtagaggactttggaaattttctctgaaaagttaaattccacataatagtaagactgtttgctgagagaaaactgacaagtaaaaactggtttaagagacagacattcaagacaaactgtattggaaatacaataatgaattttggcctgatagccctcatgctgtcttatagcaaaacactaaaattcatgcaacagagaaattggtgacatgaggactttttctccagacttcctggggaaaaactgtgagaatatacttttttcttctgtttgctttcgaaatgcattctttcttttgctgactttcccaaactttcccagtcgtttctgatgaaaaattcttcaataggaaaagaccaggtaaacttacatgaaagacatcaagtatcttttgagctccttctctctgccagaggagcaatcaactggattacacaaaactaccttcacaactaaaacaggtagaattggaacaggaattagttgtcattaatatactcgtaataaaataaagcttgttctgaaaccacaaggggtggtaagaagagactgtataaaagctactgggttctctagaaaatggatacagtatacagaatgtgagaagatacagaactcacactccagttataaaaatagacatggttctcagacaaaaagcaaatgagtacaaaagaattctccaaacgtgaactatttttaaaagatacatctatataaaacaacaagatgtcatctcagagctccaaagagtagtttgttgaaatggctgaaaaggggagatgaattggagacagataggtcaagaacccagaacagatgtgtcctactcttgtgtttggcagtgtacattggaggtcacaggcagatagactgcttttggtaatacatatataaataataatggctgactggttgatggtgcttgatggatgaatgagaaaacccaggttatcaaataatctcggtagttgaactgttagcttcttcacttgacaatgttgcacatcagaaatgattctaggttttttttacccagaatgatccctgccattcacaactcatgctccacgccccatggtttctattgtgccctaaaagatcagcctagactaatacataaatagaaaataactctggccttgaaatgaggggcagacaagtacttcatgctcagtacttataaatcacaaagaaatgctgaaattaatggtctgtctccttttactacaaaggagatgccatgagttaaagtcatgaaacaaagaaagtcaaaaagatatgggtagcagcacctttccatacccgcctggattttcaaggagcttttcactccttatgcctttcaaacaaaagttcatcagtttgaagaaaaagaaatggctctaaagttaaagagtccccagagaaaactaacagtacatgaaataggccctatgtgggcaaaaggacaagctgcagaaccagttaagacagaagaggcagcccaaggtcttactaaattacagttttagcatagtgtagcacaacatgggcagccctttttccatccaagcaacaattcagcaccatccacgtctggttcaaaagattactgaagtctgggctttcatctttggtaccacctcatgagttattcttggtttgcagtaggttcaaagaaacagaaaagctggtacctttgccttgtctgtgagtacaaacgctgggactctgattgctgcaaccattgaggccaattaaaataatactgtaacacacaggaatgatgcatccaattcctaatttccagataatagcagccatgcccctacagaggcgggatcatccatccccatcgtttaaggccttcggtttgttgtcctcagagtagaatagaacactgtgttcccacggacaaggaactccagatgaacccatggtctacatttggacagaattttaagtaccagatatgccaggcacagaaagaggactgacctgtggccatcatgcttggagaagcttctgttttggcacacaaactagaaacttcttagtgtattctggttttagttccctttcctgagtgaagcagccagggagtgaccaggttccataagccctcaatctgatacttggcattaattctctccatggtcttcttccacccaagctacaattttcccttcccatccagggatggcatcatcatcatggaaaatctcctctttgacagtgccaaactcaggatccagtgctttgaagtgataccggtgatttccttcccgatcaatagctgctttaaaatcctttaacgtcacctcctccaacctctttggtatattgaccatgaagggcgtaagtgaccggtcagtgaaatagagcactttagtacaggtgctgctgacagttggagagctctgtgagtgaggcaactttgagttagggggccaggactcccggtattcactacctacttgagttctgggtgacttgacccgaacctttctttcttgtttcttctgcgtctccataacatgcaggcgctccatgaggctagaaatgccctgctccaagctgtcaatagtgtggtgctgaggatcgtggccactgaagctgttgcgcaggctgcggagagcatctcgaacaagctgcaggtcgctggtccctctgttgctgactgaagtagctccttttcctgccgttggaaggagaaaaccattgctttgagagttgtgactgttgtagttggtcgcctcatctgcctctcttttcatacagtgagccaagaggacatctttgtgttctagctctcgctctagatccacctggtggtaactgacatcagagagtttccggagtgcttcttctaacttggcctggtgctgctgaagaaggcgatccttctgccccagctcttttttatattctcccaagagccggttcctctcatctagcttcctctgcagatccacattctggttgtgcagctcatctttgtccatatttgccctcagtagctcttgtttgagctgaagaacagatgtgtcctgctgagtcaatctctgctgcaaggcatcctttatcccctgtaagtttctggcttcttgtttacatttcagcagttccttctttaagtcctgattctcctccatactctgatccagacgactttggattataatcagttgttcctcgggattgacacctggttcacagagggccaagggcctctcctgttcatcttcaggtaaggatccattgagcagtaaggcctgtagtcctgatatcattttctttgcttcctccatttctttttctaaatattcttgttgttccaacagctgttcttcccatgaggtctccagataggttccagggctccctggccgccagtctcgagataatggagaatctgtcccttctgttctgttctctattccttcagcgggaataatcacaaaatctgccttctcttctgactgggttataatggactcgctctttgcactgtggattggactgggtgaagtcaggcttctccactctgagccctcccttggtggacgaggggtcggtcggacaggtcaggcccgcatggggctctggccgctcctcggggtggagactctga

SEQ ID NO: 16822 - RNA, 2095 nt, Homo sapiens
  source 1..2095: mol_type = other RNA
tacgtagatatatatgtattttatccgtgttgaaaatagaggaaggagaaagaatggaagacaacttgtatagtttgttatctctaaagcatctacatcttgttgcttgggagggtctccagtagatgtgccagctggggcttcaagatcagaatttgcatttaggaagttcactttcatggggtttatccatctgtgttaaaatggtagctgttcttgagggtgaggtggactcccacaggtaggtctcggcggtgcccttccatgctgtcttcattagctctggttcccttgaaactttgtggccaagaatcaggtgaaatctttcttgatgactcaggtgggcagtgttcaggatgagctgtggtgggaggaacttcatggattgactacactttgaggtcagcatggttgggttatcaaattgcagaatcagcagctttatccttttgattcaccaggagcaatcacacattgtagagtcacacaatcctgtttcttctgcttgggcacatagggagactatattccacagcctcacttgcagttaggtgaaacaatgtgattgagttctacccaggtgaatgtgggcagaagtgatatatgccacttgtagatatacccaaaaaatgtctcaggtgctggaagtgaaggacttcgcaatggaggagaaacacagtagaaggatcctggatacataagtcaccacatggaagacagccaccaggagagatgcctgactcacattggacataaatgaaatcccaagttctgatagtggtttccatgatctgtgcccctgcttcatgagaagaggaacttagtctgttttgttctgttttgtttaatgctgtgttcccagcaagaatgctgcctggcacacattaggattgactaaatatttattgaatgatggacatagaggtagagactctgctttatgtcatccttcaggttctagcttaaatgtctcttctcagagaaaccatccctgaccactatctaaagtaggcagcctctacctggtaattctccttcatagagtcctcttgttttcctttgcagcacttatcaatgatctgtaatcacatattggtttcttgccatttattcaatgttacctatcttcccagagtgtaagccccttgaggtcaggaccatgtctattttgtcacaatgggatgcctagtgcttgacttcagtagacactccatagtagacgctgcataggtattcggtggatacgagagtgaaacagtgaatgaaggaaggtggacctgggccaaggagctgggcggccaaggtcaggtttatgccatcagccccactcaggacaaatgtcccgactcctgctcggagccctcttcctactactctgtgcttcccacagctgttgatcatctcactgacaagcaggctcagccaagaaagtggaaagaggaaaagaaaaatgaggcacaggagggtagaatggaaaatctcagctcttttagcagccactcttccttatttcttgctagagtattggcacctttaaaagccttggctgtcctccccaacctccccactcaatcacaaaccgcagcacctagaaaaaaataaaggcaaaaatcaatgtgctaaatctcagttgggctcagtagcaactccctgcagcttccctctgcaagccatggaactgagctctccagccctctccctgaacttgactgcagggttggggaacttgcatgctaaaaatatgccctctccccttcggcaacccattcccaacctggtgaagaccaaggaggaagcttctgagattctcctccttgccttccatttgcagctcagattctctgtccaatgacttcatctaccctctcctgctgtccactctctgctccctttcttctcagccctcacttggtctctgccctacttacccagccagtggcctctaaagttttccattcagaatttccctctttaccttctcttttagatatgtagaaagtgaaagggaaaaggggattgttatctgggtacagacggttgagttgggaagagaatcatattttgattattaaaatattaaaatgatacagtttca

SEQ ID NO: 16823 - RNA, 2004 nt, Homo sapiens
  source 1..2004: mol_type = other RNA
tacgtagatatatatgtattttatccgtgttgaaaatagaggaaggagaaagaatggaagacaacttgtatagtttgttatctctaaagcatctacatcttgttgcttgggagggtctccagtagatgtgccagctggggcttcaagatcagaatttgcatttaggaagttcactttcatggggtttatccatctgtgttaaaatggtagctgttcttgagggtgaggtggactcccacaggtaggtctcggcggtgcccttccatgctgtcttcattagctctggttcccttgaaactttgtggccaagaatcaggtgaaatctttcttgatgactcaggtgggcagtgttcaggatgagctgtggtgggaggaacttcatggattgactacactttgaggtcagcatggttgggttatcaaattgcagaatcagcagctttatccttttgattcaccaggagcaatcacacattgtagagtcacacaatcctgtttcttctgcttgggcacatagggagactatattccacagcctcacttgcagttaggtgaaacaatgtgattgagttctacccaggtgaatgtgggcagaagtgatatatgccacttgtagatatacccaaaaaatgtctcaggtgctggaagtgaaggacttcgcaatggaggagaaacacagtagaaggatcctggatacataagtcaccacatggaagacagccaccaggagagatgcctgactcacattggacataaatgaaatcccaagttctgatagtggtttccatgatctgtgcccctgcttcatgagaagaggaacttagtctgttttgttctgttttgtttaatgctgtgttcccagcaagaatgctgcctggcacacattaggattgactaaatatttattgaatgatggacatagaggtagagactggtaattctccttcatagagtcctcttgttttcctttgcagcacttatcaatgatctgtaatcacatattggtttcttgccatttattcaatgttacctatcttcccagagtgtaagccccttgaggtcaggaccatgtctattttgtcacaatgggatgcctagtgcttgacttcagtagacactccatagtagacgctgcataggtattcggtggatacgagagtgaaacagtgaatgaaggaaggtggacctgggccaaggagctgggcggccaaggtcaggtttatgccatcagccccactcaggacaaatgtcccgactcctgctcggagccctcttcctactactctgtgcttcccacagctgttgatcatctcactgacaagcaggctcagccaagaaagtggaaagaggaaaagaaaaatgaggcacaggagggtagaatggaaaatctcagctcttttagcagccactcttccttatttcttgctagagtattggcacctttaaaagccttggctgtcctccccaacctccccactcaatcacaaaccgcagcacctagaaaaaaataaaggcaaaaatcaatgtgctaaatctcagttgggctcagtagcaactccctgcagcttccctctgcaagccatggaactgagctctccagccctctccctgaacttgactgcagggttggggaacttgcatgctaaaaatatgccctctccccttcggcaacccattcccaacctggtgaagaccaaggaggaagcttctgagattctcctccttgccttccatttgcagctcagattctctgtccaatgacttcatctaccctctcctgctgtccactctctgctccctttcttctcagccctcacttggtctctgccctacttacccagccagtggcctctaaagttttccattcagaatttccctctttaccttctcttttagatatgtagaaagtgaaagggaaaaggggattgttatctgggtacagacggttgagttgggaagagaatcatattttgattattaaaatattaaaatgatacagtttca

SEQ ID NO: 16824 - RNA, 1834 nt, Homo sapiens
  source 1..1834: mol_type = other RNA
tacgtagatatatatgtattttatccgtgttgaaaatagaggaaggagaaagaatggaagacaacttgtatagtttgttatctctaaagcatctacatcttgttgcttgggagggtctccagtagatgtgccagctggggcttcaagatcagaatttgcatttaggaagttcactttcatggggtttatccatctgtgttaaaatggtagctgttcttgagggtgaggtggactcccacaggtaggtctcggcggtgcccttccatgctgtcttcattagctctggttcccttgaaactttgtggccaagaatcaggtgaaatctttcttgatgactcaggtgggcagtgttcaggatgagctgtggtgggaggaacttcatggattgactacactttgaggtcagcatggttgggttatcaaattgcagaatcagcagctttatccttttgattcaccaggagcaatcacacattgtagagtcacacaatcctgtttcttctgcttgggcacatagggagactatattccacagcctcacttgcagttaggtgaaacaatgtgattgagttctacccaggtgaatgtgggcagaagtgatatatgccacttgtagatatacccaaaaaatgtctcaggtgctggaagtgaaggacttcgcaatggaggagaaacacagtagaaggatcctggatacataagtcaccacatggaagacagccaccaggagagatgcctgactcacattggacattttagaggccagaagtcaggaatcaaggtatctgcaaggccaggctccctctgatacctgcacaggagaatactcgcccccatcaagcctctggtgtttgctggcagtgcttggcatccctcagctgatcgatgcgtcagtcccacttctgcctccatggtcagcaggcatcctcccctcgtgtgtctgtgtctccatgtggtattctcctgcccatgtgtctttctccctgcctctgctttgtagttacaggcaaacaggggctgggaaggtgaagagtggatgtctgaacaaaatttaattcctgttaggaaagaagaaaggggcaatggatgttaggtaaggagataaaatgtacaatacactttaatgatacaacataacagttacgaaagaagctaagaatggtgaagggggctccacttacctttggtttatttattccaccagtcttccttccttcctttttgttttacacctgtaagcttcagactctagagtggtgggttcaccaaccactccaaatcctacccctgcaatggattttattataccaccaggttgagtgaagctgaccaacttcaggggcttcagggaggtggtaaaggcagggaggggataactgagaggtgagagtcacacagtgcccactttctaggtaatcaattgacagcaattcagcatgccatcattgctgttctagctgtatgtagttgatgtacacaactgagagggaggttgcaagtatgagaattttttatacacatataaaaaattatatatctctatatatcttgtcaatgagcaaaaaattgaaatgtgagactaccttaaaccttgattctttctctcgtcttatgttcttgaacactcttccacagtagggggcaatctgactggagagtgaaatactctttcttgttgaatgaccatggcactcctgtcttagtttcttctcaccctatttctaggccaaggtcatttccctgtaacatccttaataacggattctgagcccagaccaggcacggtggctcatgcctgtaatcccagcactttgggaggctgagacaggcggat

SEQ ID NO: 16825 - RNA, 1223 nt, Homo sapiens
  source 1..1223: mol_type = other RNA
tacgtagatatatatgtattttatccgtgttgaaaatagaggaaggagaaagaatggaagacaacttgtatagtttgttatctctaaagcatctacatcttgttgcttgggagggtctccagtagatgtgccagctggggcttcaagatcagaatttgcatttaggaagttcactttcatggggtttatccatctgtgttaaaatggtagctgttcttgagggtgaggtggactcccacaggtaggtctcggcggtgcccttccatgctgtcttcattagctctggttcccttgaaactttgtggccaagaatcaggtgaaatctttcttgatgactcaggtgggcagtgttcaggatgagctgtggtgggaggaacttcatggattgactacactttgaggtcagcatggttgggttatcaaattgcagaatcagcagctttatccttttgattcaccaggagcaatcacacattgtagagtcacacaatcctgtttcttctgcttgggcacatagggagactatattccacagcctcacttgcagttaggtgaaacaatgtgattgagttctacccaggtgaatgtgggcagaagtgatatatgccacttgtagatatacccaaaaaatgtctcaggtgctggaagtgaaggacttcgcaatggaggagaaacacagtagaaggatcctggatacataagtcaccacatggaagacagccaccaggagagatgcctgactcacattggacattttagaggccagaagtcaggaatcaaggtatctgcaaggccaggctccctctgatacctgcacaggagaatactcgcccccatcaagcctctggtgtttgctggcagtgcttggcatccctcagctgatcgatgcgtcagtcccacttctgcctccatggtcagcaggcatcctcccctcgtgtgtctgtgtctccatgtggtattctcctgcccatgtgtctttctccctgcctctgctttgtagttacaggcaaacaggggctgggaaggtgaagagtggatgtctgaacaaaatttaattccttggcaggcttcccatcaaatattgttgcgcaaaggatggatggatgaaaggaagagtgagccaataaacgagggaacgccgggaaaggcagcctcaagccggtgggccctgccacccccaccgtccctgagcatccgagccggttcccgcccccggcccgaac

SEQ ID NO: 16826 - RNA, 1325 nt, Homo sapiens
  source 1..1325: mol_type = other RNA
tacgtagatatatatgtattttatccgtgttgaaaatagaggaaggagaaagaatggaagacaacttgtatagtttgttatctctaaagcatctacatcttgttgcttgggagggtctccagtagatgtgccagctggggcttcaagatcagaatttgcatttaggaagttcactttcatggggtttatccatctgtgttaaaatggtagctgttcttgagggtgaggtggactcccacaggtaggtctcggcggtgcccttccatgctgtcttcattagctctggttcccttgaaactttgtggccaagaatcaggtgaaatctttcttgatgactcaggtgggcagtgttcaggatgagctgtggtgggaggaacttcatggattgactacactttgaggtcagcatggttgggttatcaaattgcagaatcagcagctttatccttttgattcaccaggagcaatcacacattgtagagtcacacaatcctgtttcttctgcttgggcacatagggagactatattccacagcctcacttgcagttaggtgaaacaatgtgattgagttctacccaggtgaatgtgggcagaagtgatatatgccacttgtagatatacccaaaaaatgtctcaggtgctggaagtgaaggacttcgcaatggaggagaaacacagtagaaggatcctggatacataagtcaccacatggaagacagccaccaggagagatgcctgactcacattggacattttagaggccagaagtcaggaatcaaggtatctgcaaggccaggctccctctgatacctgcacaggagaatactcgcccccatcaagcctctggtgtttgctggcagtgcttggcatccctcagctgatcgatgcgtcagtcccacttctgcctccatggtcagcaggcatcctcccctcgtgtgtctgtgtctccatgtggtattctcctgcccatgtgtctttctccctgcctctggaaccagaagacctgggttcaagtcattgccttgctgtttattagctgtgtggcctccagaagtcacttgatttctttgacctcgatgaccaatctgtgaactcagggcaattctagtcttttccatttacgatgttcttgtgagaatcaaatggagtaatctgaaaacttggcaggcttcccatcaaatattgttgcgcaaaggatggatggatgaaaggaagagtgagccaataaacgagggaacgccgggaaaggcagcctcaagccggtgggccctgccacccccaccgtccctgagcatccgagccggttcccgcccccggcccgaac

SEQ ID NO: 16827 - RNA, 1154 nt, Homo sapiens
  source 1..1154: mol_type = other RNA
tacgtagatatatatgtattttatccgtgttgaaaatagaggaaggagaaagaatggaagacaacttgtatagtttgttatctctaaagcatctacatcttgttgcttgggagggtctccagtagatgtgccagctggggcttcaagatcagaatttgcatttaggaagttcactttcatggggtttatccatctgtgttaaaatggtagctgttcttgagggtgaggtggactcccacaggtaggtctcggcggtgcccttccatgctgtcttcattagctctggttcccttgaaactttgtggccaagaatcaggtgaaatctttcttgatgactcaggtgggcagtgttcaggatgagctgtggtgggaggaacttcatggattgactacactttgaggtcagcatggttgggttatcaaattgcagaatcagcagctttatccttttgattcaccaggagcaatcacacattgtagagtcacacaatcctgtttcttctgcttgggcacatagggagactatattccacagcctcacttgcagttaggtgaaacaatgtgattgagttctacccaggtgaatgtgggcagaagtgatatatgccacttgtagatatacccaaaaaatgtctcaggtgctggaagtgaaggacttcgcaatggaggagaaacacagtagaaggatcctggatacataagtcaccacatggaagacagccaccaggagagatgcctgactcacattggacattttagaggccagaagtcaggaatcaaggtatctgcaaggccaggctccctctgatacctgcacaggagaatactcgcccccatcaagcctctggtgtttgctggcagtgcttggcatccctcagctgatcgatgcgtcagtcccacttctgcctccatggtcagcaggcatcctcccctcgtgtgtctgtgtctccatgtggtattctcctgcccatgtgtctttctccctgcctcttggcaggcttcccatcaaatattgttgcgcaaaggatggatggatgaaaggaagagtgagccaataaacgagggaacgccgggaaaggcagcctcaagccggtgggccctgccacccccaccgtccctgagcatccgagccggttcccgcccccggcccgaac

SEQ ID NO: 16828 - RNA, 1915 nt, Homo sapiens
  source 1..1915: mol_type = other RNA
tacgtagatatatatgtattttatccgtgttgaaaatagaggaaggagaaagaatggaagacaacttgtatagtttgttatctctaaagcatctacatcttgttgcttgggagggtctccagtagatgtgccagctggggcttcaagatcagaatttgcatttaggaagttcactttcatggggtttatccatctgtgttaaaatggtagctgttcttgagggtgaggtggactcccacaggtaggtctcggcggtgcccttccatgctgtcttcattagctctggttcccttgaaactttgtggccaagaatcaggtgaaatctttcttgatgactcaggtgggcagtgttcaggatgagctgtggtgggaggaacttcatggattgactacactttgaggtcagcatggttgggttatcaaattgcagaatcagcagctttatccttttgattcaccaggagcaatcacacattgtagagtcacacaatcctgtttcttctgcttgggcacatagggagactatattccacagcctcacttgcagttaggtgaaacaatgtgattgagttctacccaggtgaatgtgggcagaagtgatatatgccacttgtagatatacccaaaaaatgtctcaggtgctggaagtgaaggacttcgcaatggaggagaaacacagtagaaggatcctggatacataagtcaccacatggaagacagccaccaggagagatgcctgactcacattggactctgctttatgtcatccttcaggttctagcttaaatgtctcttctcagagaaaccatccctgaccactatctaaagtaggcagcctctacctggtaattctccttcatagagtcctcttgttttcctttgcagcacttatcaatgatctgtaatcacatattggtttcttgccatttattcaatgttacctatcttcccagagtgtaagccccttgaggtcaggaccatgtctattttgtcacaatgggatgcctagtgcttgacttcagtagacactccatagtagacgctgcataggtattcggtggatacgagagtgaaacagtgaatgaaggaaggtggacctgggccaaggagctgggcggccaaggtcaggtttatgccatcagccccactcaggacaaatgtcccgactcctgctcggagccctcttcctactactctgtgcttcccacagctgttgatcatctcactgacaagcaggctcagccaagaaagtggaaagaggaaaagaaaaatgaggcacaggagggtagaatggaaaatctcagctcttttagcagccactcttccttatttcttgctagagtattggcacctttaaaagccttggctgtcctccccaacctccccactcaatcacaaaccgcagcacctagaaaaaaataaaggcaaaaatcaatgtgctaaatctcagttgggctcagtagcaactccctgcagcttccctctgcaagccatggaactgagctctccagccctctccctgaacttgactgcagggttggggaacttgcatgctaaaaatatgccctctccccttcggcaacccattcccaacctggtgaagaccaaggaggaagcttctgagattctcctccttgccttccatttgcagctcagattctctgtccaatgacttcatctaccctctcctgctgtccactctctgctccctttcttctcagccctcacttggtctctgccctacttacccagccagtggcctctaaagttttccattcagaatttccctctttaccttctcttttagatatgtagaaagtgaaagggaaaaggggattgttatctgggtacagacggttgagttgggaagagaatcatattttgattattaaaatattaaaatgatacagtttca

SEQ ID NO: 16829 - RNA, 3242 nt, Homo sapiens
  source 1..3242: mol_type = other RNA
tacgtagatatatatgtattttcctaagataaaactcttctcagaatttcattactttttattatacaccaactagtttatattgtagttctttacaaagaaaatgctaagaaaaattataatcacatgttatatggttttaaaataataattccagatttctttacatataagatggaatggtccagcagctatatccactgtcacagactttagttccgttcaatgatatggcacatcctgcaaaattaactagtcacacacaaaaaatgtctcaaatacagtaaaaatgtacacacaaaggtaatttacaatgacaaggaatgtaatttttcttggctgtgcttcagaaatttagggtcagtagccttaatcaaggcacaaagcaggaaaaggtgagcacagctgtctctaggagtgggcaaggtatgtacaatcactgatgaggtatgcatgcacgcaaaggatttaaaactgctcagtctcactacaaaaattgaactgagttaaaaggaaatgctgtggcttccccctactatctggctctggattgagtccacagtcttacttcatcaaatagaaaataaaactgacaaggatctccaaaagtaaatcactatttgtgtaaatgaaacaaaatgcttcattaatcccagttcttggttgtgcctcctggactagaagcattttgtagacaaaagagtgtttcacaaaattgaaatgtaattcaggtgaaggacaaaacattttccacagacacttaaaattccaaactttcaaatggcccttacagctgaaccgttgtatgttacagtagtgagggttctgggtatcctttagcagcaaatgccggtttaaagggcacggggtctcttcgggttgatttgcttgctggcttgttcctcctcttgtagagctgcacggaaagatttcactttatcccgcagttcagttaaaatgtctattttttgctcaagaatagcttcaagttgtgtagcatatgaatcgacatcataatctacttcttcagtcatctctaagagggccttttcatcttctaaccaccgaatagattcctggaacactgccctgtgatcttctacaacttgttcttccatttctaccatttgtgaaacagcttcgtggaaagtaaacaactgtggagagacttcttcttcattttgttcacaaagaagttttagatcatctctctgaggggaactccccacaccccactgtgtctctaagtcatcaatctggtttggtggatggtgcattattggacgaacatcaccagcagcagttggatctacagtcaattctttgaccctatttgcatatcttaatgtattaagagtattttcacaggatgccattcctggagagattgtggcaatcatgcaggtacgagagttttcacctatgaaagaatctcttaacacctgagtgagtttacttgcacggaaaggagtatgaggtttatttctacctaaggctctgatgcactccttgagtgctaaaaggcttttattaatttcagcaccttcaagcctagtttgcctgtccgcactggaagtatcagctcctctttcatttccagccaaatcaatgagagaaaatttgccatgtagttttcctttccttctaagaataatctgaaacactgcatggctccgagatgaatgtgcatttgcagatgtttgaccggatgttctgcaactgttgcctatgtcaatgagtttcagtacatcttcaacacatttgacctcccgttcctgtaatcccaccacttgaacctgctgttttccatcttctagaactcttaattttgttttcctgtttagcaagtcaaacacctttccactataaatttcaaagaaggttgcatatacttgaagttctagcttcttatagtttggcttctttagcattaaaaagacatctcgagctgctaatgcataaattcctttagaacaatcttggttctttcctgaaaagtcaccacccatagtatgagtttttccacttccagtctgcccataagcaaagcatgtagccattcccctttcaaatatagtttccactagtggtctagcagtaaacctgtaaaccatttcattaggagctgagtcatcaaaggcataatcaaaacgaaatgtttggttttctaggtaccttgttaaatctactttttgttttggttcatgtaccatcacaacatctttactaggaattgtgattacatcaagatctttcatttgagtttcttttttattgagtggtcgttttcttacacacacacatatcctatgttcatcaataggatctgctgttgttaatggtctataatccaaacttcctctaaagtctctgatcatacacataatttcataatttgggtttgtagcatcaacgtcctgggctcttttttctctaagttcttgctgttgcaatctccttttctctcgtttttcttgcagtttttctacttctttcacacaattagattttctacgtgaagggggtccaaattccttttttgcagcttgaactggagatatatctgaaacactaccattctgttgtgcagaggaagactgttcaggaaattgactgggccgtgcacgtgctgaaccaaccactctattatctcttgaaggagggtcattcttaatagaagctacagtccgtcgattctttacaattttgtttactttggctgaggatgctggaggtggaggtgtttctggactgggttcaatttcttcatcaggaacaaggtcagggttaagtgaaaagatgctctccaggtcaatctctttgccttttgtatctccattttctatccattcaacagttacactttcattatcttcatttaaagatgttaccattgcttgatgtattcggccatcgctgcgcttgatctccacgtaaatcccgatctggatcttgccgaagttggccgttgccatcacctcatctggagcagcagcagcgggccgagggagggggaccggagggcggaaaaggcggggagggggcggggtaggtgtgggagggggagcggttgcccgcggccgcgccggcccgggcgacagcgtgaacgcaagcggggccgcaaggagcagctgtggggaagcaggcggaggccccgggcctgcaggccggcaggaggacgcgcacgccgggtagtcggggtgaagctagggccggggccgtgagacggcgcggggtagagt

SEQ ID NO: 16830 - RNA, 3445 nt, Homo sapiens
  source 1..3445: mol_type = other RNA
tacgtagatatatatgtattttcctaagataaaactcttctcagaatttcattactttttattatacaccaactagtttatattgtagttctttacaaagaaaatgctaagaaaaattataatcacatgttatatggttttaaaataataattccagatttctttacatataagatggaatggtccagcagctatatccactgtcacagactttagttccgttcaatgatatggcacatcctgcaaaattaactagtcacacacaaaaaatgtctcaaatacagtaaaaatgtacacacaaaggtaatttacaatgacaaggaatgtaatttttcttggctgtgcttcagaaatttagggtcagtagccttaatcaaggcacaaagcaggaaaaggtgagcacagctgtctctaggagtgggcaaggtatgtacaatcactgatgaggtatgcatgcacgcaaaggatttaaaactgctcagtctcactacaaaaattgaactgagttaaaaggaaatgctgtggcttccccctactatctggctctggattgagtccacagtcttacttcatcaaatagaaaataaaactgacaaggatctccaaaagtaaatcactatttgtgtaaatgaaacaaaatgcttcattaatcccagttcttggttgtgcctcctggactagaagcattttgtagacaaaagagtgtttcacaaaattgaaatgtaattcaggtgaaggacaaaacattttccacagacacttaaaattccaaactttcaaatggcccttacagctgaaccgttgtatgttacagtagtgagggttctgggtatcctttagcagcaaatgccggtttaaagggcacggggtctcttcgggttgatttgcttgctggcttgttcctcctcttgtagagctgcacggaaagatttcactttatcccgcagttcagttaaaatgtctattttttgctcaagaatagcttcaagttgtgtagcatatgaatcgacatcataatctacttcttcagtcatctctaagagggccttttcatcttctaaccaccgaatagattcctggaacactgccctgtgatcttctacaacttgttcttccatttctaccatttgtgaaacagcttcgtggaaagtaaacaactgtggagagacttcttcttcattttgttcacaaagaagttttagatcatctctctgaggggaactccccacaccccactgtgtctctaagtcatcaatctggtttggtggatggtgcattattggacgaacatcaccagcagcagttggatctacagtcaattctttgaccctatttgcatatcttaatgtattaagagtattttcacaggatgccattcctggagagattgtggcaatcatgcaggtacgagagttttcacctatgaaagaatctcttaacacctgagtgagtttacttgcacggaaaggagtatgaggtttatttctacctaaggctctgatgcactccttgagtgctaaaaggcttttattaatttcagcaccttcaagcctagtttgcctgtccgcactggaagtatcagctcctctttcatttccagccaaatcaatgagagaaaatttgccatgtagttttcctttccttctaagaataatctgaaacactgcatggctccgagatgaatgtgcatttgcagatgtttgaccggatgttctgcaactgttgcctatgtcaatgagtttcagtacatcttcaacacatttgacctcccgttcctgtaatcccaccacttgaacctgctgttttccatcttctagaactcttaattttgttttcctgtttagcaagtcaaacacctttccactataaatttcaaagaaggttgcatatacttgaagttctagcttcttatagtttggcttctttagcattaaaaagacatctcgagctgctaatgcataaattcctttagaacaatcttggttctttcctgaaaagtcaccacccatagtatgagtttttccacttccagtctgcccataagcaaagcatgtagccattcccctttcaaatatagtttccactagtggtctagcagtaaacctgtaaaccatttcattaggagctgagtcatcaaaggcataatcaaaacgaaatgtttggttttctaggtaccttgttaaatctactttttgttttggttcatgtaccatcacaacatctttactaggaattgtgattacatcaagatctttcatttgagtttcttttttattgagtggtcgttttcttacacacacacatatcctatgttcatcaataggatctgctgttgttaatggtctataatccaaacttcctctaaagtctctgatcatacacataatttcataatttgggtttgtagcatcaacgtcctgggctcttttttctctaagttcttgctgttgcaatctccttttctctcgtttttcttgcagtttttctacttctttcacacaattagattttctacgtgaagggggtccaaattccttttttgcagcttgaactggagatatatctgaaacactaccattctgttgtgcagaggaagactgttcaggaaattgactgggccgtgcacgtgctgaaccaaccactctattatctcttgaaggagggtcattcttaatagaagctacagtccgtcgattctttacaattttgtttactttggctgaggatgctggaggtggaggtgtttctggactgggttcaatttcttcatcaggaacaaggtcagggttaagtgaaaagatgctctccaggtcaatctctttgccttttgtatctccattttctatccattcaacagttacactttcattatcttcatttaaagatgttaccattgcttgatgtattcggcccatcgatggacatttaggttgcttccctatcttggctactgtgaataatgctgcaatgaacgcgagagtgcagatatcttcacaaggtggtgatttcctctcccttgggtgtataccagggacaggtgttgctgtgcacccagaatcttcaaaataatatgtaaatcctacttttgctggtatactgtgaactcgtatttaccatcgctgcgcttgatctccacgtaaatcccgatctggatcttgccgaagttggccgttgccatcacctcatctggagcagcagcagcgggccgagggagggggaccggagggcggaaaaggcggggagggggcggggtaggtgtgggagggggagcggttgcccgcggccgcgccggcccgggcgacagcgtgaacgcaagcggggccgcaaggagcagctgtggggaagcaggcggaggccccgggcctgcaggccggcaggaggacgcgcacgccgggtagtcggggtgaagctagggccggggccgtgagacggcgcggggtagagt

SEQ ID NO: 16831 - RNA, 3185 nt, Homo sapiens
  source 1..3185: mol_type = other RNA
tacgtagatatatatgtattttcctaagataaaactcttctcagaatttcattactttttattatacaccaactagtttatattgtagttctttacaaagaaaatgctaagaaaaattataatcacatgttatatggttttaaaataataattccagatttctttacatataagatggaatggtccagcagctatatccactgtcacagactttagttccgttcaatgatatggcacatcctgcaaaattaactagtcacacacaaaaaatgtctcaaatacagtaaaaatgtacacacaaaggtaatttacaatgacaaggaatgtaatttttcttggctgtgcttcagaaatttagggtcagtagccttaatcaaggcacaaagcaggaaaaggtgagcacagctgtctctaggagtgggcaaggtatgtacaatcactgatgaggtatgcatgcacgcaaaggatttaaaactgctcagtctcactacaaaaattgaactgagttaaaaggaaatgctgtggcttccccctactatctggctctggattgagtccacagtcttacttcatcaaatagaaaataaaactgacaaggatctccaaaagtaaatcactatttgtgtaaatgaaacaaaatgcttcattaatcccagttcttggttgtgcctcctggactagaagcattttgtagacaaaagagtgtttcacaaaattgaaatgtaattcaggtgaaggacaaaacattttccacagacacttaaaattccaaactttcaaatggcccttacagctgaaccgttgtatgttacagtagtgagggttctgggtatcctttagcagcaaatgccggtttaaagggcacggggtctcttcgggttgatttgcttgctggcttgttcctcctcttgtagagctgcacggaaagatttcactttatcccgcagttcagttaaaatgtctattttttgctcaagaatagcttcaagttgtgtagcatatgaatcgacatcataatctacttcttcagtcatctctaagagggccttttcatcttctaaccaccgaatagattcctggaacactgccctgtgatcttctacaacttgttcttccatttctaccatttgtgaaacagcttcgtggaaagtaaacaactgtggagagacttcttcttcattttgttcacaaagaagttttagatcatctctctgaggggaactccccacaccccactgtgtctctaagtcatcaatctggtttggtggatggtgcattattggacgaacatcaccagcagcagttggatctacagtcaattctttgaccctatttgcatatcttaatgtattaagagtattttcacaggatgccattcctggagagattgtggcaatcatgcaggtacgagagttttcacctatgaaagaatctcttaacacctgagtgagtttacttgcacggaaaggagtatgaggtttatttctacctaaggctctgatgcactccttgagtgctaaaaggcttttattaatttcagcaccttcaagcctagtttgcctgtccgcactggaagtatcagctcctctttcatttccagccaaatcaatgagagaaaatttgccatgtagttttcctttccttctaagaataatctgaaacactgcatggctccgagatgaatgtgcatttgcagatgtttgaccggatgttctgcaactgttgcctatgtcaatgagtttcagtacatcttcaacacatttgacctcccgttcctgtaatcccaccacttgaacctgctgttttccatcttctagaactcttaattttgttttcctgtttagcaagtcaaacacctttccactataaatttcaaagaaggttgcatatacttgaagttctagcttcttatagtttggcttctttagcattaaaaagacatctcgagctgctaatgcataaattcctttagaacaatcttggttctttcctgaaaagtcaccacccatagtatgagtttttccacttccagtctgcccataagcaaagcatgtagccattcccctttcaaatatagtttccactagtggtctagcagtaaacctgtaaaccatttcattaggagctgagtcatcaaaggcataatcaaaacgaaatgtttggttttctaggtaccttgttaaatctactttttgttttggttcatgtaccatcacaacatctttactaggaattgtgattacatcaagatctttcatttgagtttcttttttattgagtggtcgttttcttacacacacacatatcctatgttcatcaataggatctgctgttgttaatggtctataatccaaacttcctctaaagtctctgatcatacacataatttcataatttgggtttgtagcatcaacgtcctgggctcttttttctctaagttcttgctgttgcaatctccttttctctcgtttttcttgcagtttttctacttctttcacacaattagattttctacgtgcattctgttgtgcagaggaagactgttcaggaaattgactgggccgtgcacgtgctgaaccaaccactctattatctcttgaaggagggtcattcttaatagaagctacagtccgtcgattctttacaattttgtttactttggctgaggatgctggaggtggaggtgtttctggactgggttcaatttcttcatcaggaacaaggtcagggttaagtgaaaagatgctctccaggtcaatctctttgccttttgtatctccattttctatccattcaacagttacactttcattatcttcatttaaagatgttaccattgcttgatgtattcggccatcgctgcgcttgatctccacgtaaatcccgatctggatcttgccgaagttggccgttgccatcacctcatctggagcagcagcagcgggccgagggagggggaccggagggcggaaaaggcggggagggggcggggtaggtgtgggagggggagcggttgcccgcggccgcgccggcccgggcgacagcgtgaacgcaagcggggccgcaaggagcagctgtggggaagcaggcggaggccccgggcctgcaggccggcaggaggacgcgcacgccgggtagtcggggtgaagctagggccggggccgtgagacggcgcggggtagagt

SEQ ID NO: 16832 - RNA, 3356 nt, Homo sapiens
  source 1..3356: mol_type = other RNA
tacgtagatatatatgtattttcctaagataaaactcttctcagaatttcattactttttattatacaccaactagtttatattgtagttctttacaaagaaaatgctaagaaaaattataatcacatgttatatggttttaaaataataattccagatttctttacatataagatggaatggtccagcagctatatccactgtcacagactttagttccgttcaatgatatggcacatcctgcaaaattaactagtcacacacaaaaaatgtctcaaatacagtaaaaatgtacacacaaaggtaatttacaatgacaaggaatgtaatttttcttggctgtgcttcagaaatttagggtcagtagccttaatcaaggcacaaagcaggaaaaggtgagcacagctgtctctaggagtgggcaaggtatgtacaatcactgatgaggtatgcatgcacgcaaaggatttaaaactgctcagtctcactacaaaaattgaactgagttaaaaggaaatgctgtggcttccccctactatctggctctggattgagtccacagtcttacttcatcaaatagaaaataaaactgacaaggatctccaaaagtaaatcactatttgtgtaaatgaaacaaaatgcttcattaatcccagttcttggttgtgcctcctggactagaagcattttgtagacaaaagagtgtttcacaaaattgaaatgtaattcaggtgaaggacaaaacattttccacagacacttaaaattccaaactttcaaatggcccttacagctgaaccgttgtatgttacagtagtgagggttctgggtatcctttagcagcaaatgccggtttaaagggcacggggtctcttcgggttgatttgcttgctggcttgttcctcctcttgtagagctgcacggaaagatttcactttatcccgcagttcagttaaaatgtctattttttgctcaagaatagcttcaagttgtgtagcatatgaatcgacatcataatctacttcttcagtcatctctaagagggccttttcatcttctaaccaccgaatagattcctggaacactgccctgtgatcttctacaacttgttcttccatttctaccatttgtgaaacagcttcgtggaaagtaaacaactgtggagagacttcttcttcattttgttcacaaagaagttttagatcatctctctgaggggaactccccacaccccactgtgtctctaagtcatcaatctggtttggtggatggtgcattattggacgaacatcaccagcagcagttggatctacagtcaattctttgaccctggtaactgaaggagaaaagtcgtcatattcataagaaggagagagatcagggcgactgccactaccctgtgagaagggaatgtctgatggactaattccaaactcctttactctatttgcatatcttaatgtattaagagtattttcacaggatgccattcctggagagattgtggcaatcatgcaggtacgagagttttcacctatgaaagaatctcttaacacctgagtgagtttacttgcacggaaaggagtatgaggtttatttctacctaaggctctgatgcactccttgagtgctaaaaggcttttattaatttcagcaccttcaagcctagtttgcctgtccgcactggaagtatcagctcctctttcatttccagccaaatcaatgagagaaaatttgccatgtagttttcctttccttctaagaataatctgaaacactgcatggctccgagatgaatgtgcatttgcagatgtttgaccggatgttctgcaactgttgcctatgtcaatgagtttcagtacatcttcaacacatttgacctcccgttcctgtaatcccaccacttgaacctgctgttttccatcttctagaactcttaattttgttttcctgtttagcaagtcaaacacctttccactataaatttcaaagaaggttgcatatacttgaagttctagcttcttatagtttggcttctttagcattaaaaagacatctcgagctgctaatgcataaattcctttagaacaatcttggttctttcctgaaaagtcaccacccatagtatgagtttttccacttccagtctgcccataagcaaagcatgtagccattcccctttcaaatatagtttccactagtggtctagcagtaaacctgtaaaccatttcattaggagctgagtcatcaaaggcataatcaaaacgaaatgtttggttttctaggtaccttgttaaatctactttttgttttggttcatgtaccatcacaacatctttactaggaattgtgattacatcaagatctttcatttgagtttcttttttattgagtggtcgttttcttacacacacacatatcctatgttcatcaataggatctgctgttgttaatggtctataatccaaacttcctctaaagtctctgatcatacacataatttcataatttgggtttgtagcatcaacgtcctgggctcttttttctctaagttcttgctgttgcaatctccttttctctcgtttttcttgcagtttttctacttctttcacacaattagattttctacgtgaagggggtccaaattccttttttgcagcttgaactggagatatatctgaaacactaccattctgttgtgcagaggaagactgttcaggaaattgactgggccgtgcacgtgctgaaccaaccactctattatctcttgaaggagggtcattcttaatagaagctacagtccgtcgattctttacaattttgtttactttggctgaggatgctggaggtggaggtgtttctggactgggttcaatttcttcatcaggaacaaggtcagggttaagtgaaaagatgctctccaggtcaatctctttgccttttgtatctccattttctatccattcaacagttacactttcattatcttcatttaaagatgttaccattgcttgatgtattcggccatcgctgcgcttgatctccacgtaaatcccgatctggatcttgccgaagttggccgttgccatcacctcatctggagcagcagcagcgggccgagggagggggaccggagggcggaaaaggcggggagggggcggggtaggtgtgggagggggagcggttgcccgcggccgcgccggcccgggcgacagcgtgaacgcaagcggggccgcaaggagcagctgtggggaagcaggcggaggccccgggcctgcaggccggcaggaggacgcgcacgccgggtagtcggggtgaagctagggccggggccgtgagacggcgcggggtagagt

SEQ ID NO: 16833 - RNA, 564 nt, Homo sapiens
  source 1..564: mol_type = other RNA
tacgtagatatatatgtattttcctttaaatatttgatatattagaggaacatgaggaaggaacagttctaaccaagagctctttgggtaacagctgtcaggtaacagtggaaggtcttagcccagaagctgggctgccttgggcaggctcccagagactaccttggcttctcttggctctgcagaaagggaacgatgagctgcttttttaaagaggcgtgccctaggttcattcatgctctttactgggcttttcagaagagtggggagttttagtttaccttcttgatgataaatccacagtataccccaagtgaccagacctttattaaagggtgtcattagcttgaagcctttccttctgttatatgctattgccttgtggtctcagaatgatcactatcgttaacattcacgggtggttcacttatcattcctgactgcacagacatggcagccgctcggaagcgtccgcaggtgtagcatggtgatacatattacattgtgccacaatggatttatgtatttttaaaacttgcttaaacacggccgggcgcggtggct

SEQ ID NO: 16834 - RNA, 7170 nt, Homo sapiens
  source 1..7170: mol_type = other RNA
tacgtagatatatatgtattttcttttccttgttagaaaaatactgtattgtcttttggtctgatggtgataggctgagataaaatttaattaacattaaattcatcaaaaatttatctcttaaaaaagcacaatatagagatattatattgtgacagaatttcttaccctagaaataatttttcaaatctcaaatattaaatattagtgttgactcatggatatatgttaaaaatatgtcctcaatctctatttttattataattttctcagttacacaagtttttgtatattggaaacgtcagttgtcaacattaaatacataaaaatgccctatataaaaaataattaacagctattcctagagtggtaaaatgtagcccaactaaaaaaaacaaagtatttgtaattagttgaaatgtcttttacctttaaattctttaacctgttattcgttgaaggttactgatttttcttattttaaatagaaataagaatattttcttattttaaataaaaagcaattattttgaaattatacccttaatagggtataaagtttctttaataagaaactttcctttaaagtgttataaccttttaatggttgaaagttatttgtttttcttattttaaataaacagtaattatgttgaaatcatatcctatcaaagaaacaacatgtttacaagtaaatacatgtataagcattaaatgctagcaggggtctccaatcttttggcttccctgggccacactggaagaaccatcttgggccacacataaaatacacgaacactaatgatagctgatgagctaaaaaataaaataaaataaaataaaataataaataaaataaaataaaataaaatcacaaaatatctcatcatgttttaagaaagcttacaaaatttgtgttggggccgcattcaaagccatcctgggctgcatgtggcctgtgggttgaacaagcttgcactaaggcaaataaaaattgttaacactgggtcagaaaattacacagaaaaatgtttaggatgactcttattatgaaacatgatttacttcctaaaattagccacggttatgtaggatgttttttctattcacttcactctatactaaaaacttcattcagtatatatttactcaatatttatcatatgacatacttataaatattatgagtatatggcaggaatgaatcctttttaaaataaggttatacacataccaatcagacactgactagagttaggacaaatactattctcatttgaaatgaggactaaagactaaaccacttgccttattgatcccagagccacaaccaaatataaaaatcttaactcccatgttaaatgtttttttctacaagcccacagttcctaagtcatatttcaatttccatttaaaaattttcaaatttatatcacaattcttacttgcttcactttttaatgaaattccaattacttcaaagataataaacgcttgctaacctaataaacacaaaatttatttcttcatgtgaataaatattttatttaaaagtgagtccaaaataacagtccactatttaggtggtataaataaaaatggtagatcccttcctctctcctctcttccaacaattctaaggaaaataatatcaagccaagtggcaattaagttcaaactagaaatacatttcattaagctacgtatttattagaaataaattacattaggctatttacacaagttattttatgactggctatgcacatttcagaaataactctaagaagacaaagaaaaggccagacagctaaaataatttatcttgccaaaatgagatgctaagtttaaactgagagatgctatctttccaaatcatttaaatacatagacgcagttcaaaagattcctgactatccattaatggaaaacataaacgttaacaaaattcacagcatacctgaatcttactcatgctacctaaagataacatatctctagaatttcacagaagatagaatcagttcaaaatgatgtattactgaacctataatgatttatggactagatatttttatgacacttttcaaaatagacatactcacagactttagtaatggtaactgtagggctccagatgccctcgagcagggcaatatttttttcataatcacctaattttaatcaattcagctaagtctaatgtttaaaaattcatgaaaaaatatctatctactcaataacttttgaaaacacaaatataactaagaatgtttctaaaagcaaggatctaaacacctaagaatggtcttctcagttgtttcaagtgaatgactttgagtttagtatcatttcttgaacgactaaaggcaaaatgatctgttgtgccaagttcttacataatcattttatctgttatctattttggaaaattcaccagcaaatggccatctttgaactgcctagaaaatttaacgaagacatttatcttaaattcgaaagtattgataagcattcctgttttaaaataataaatagttgaaaatagcaccttttaatacatggcattcttttcttaaaatgccaagtactatattttatgtattttataaaaaatgtggaagattaacctgtttctctctgaatgtagattttcaccaaaacatctcttaaacagcagggactcaacacttaaaaatgaactagaagagctgggcacagtggctcacgcctgtaatcccagcactttgggaggcgaggcaggtggattacctgaggtcaggagttcgagaccagcctggctaacacggtgaaaccccggctctactaaaaatagaaaaaattagccaggcttggtggtgggcgcctataatctcagctactcgggaggctgaggcaggagaactgcttgaacccaggaggtggaggtttcagtgagccaagatcgcgccattgcattccagcctgggggacaagagcgagacttctcctcaaagacaaaaacaaacaaaaaaagatatagaacagtgatccctccaaagagcagtcttctttaattacagggtagaatattttcctcaattttgccagactagatcagagtggaagcttctcctctcagaagtattcctaaatacaaaatccttgcattaatattatcagacaaaaagttactttccctaaattacacattcttttttcaattttgacttcccagatttagttctccactatagtaaattaatgacaaaagtataatttctttgagtgtcctctctcatctaatttttaagaagtctgggtaaaacacgtttttctacaatcactgttataactaatgccgatctattttctgagtactagagtacaaccaaaaaatggcctgcatttattactcaaattatacttgtaattttcacctgcacacaattttatatttgtaaatgtagactcatcacttaaaactcagagaagcaaaatttgacattgaggggaaagtaatttgttcacttatagctacttttaaagtttagaaacataaaattatgttaaaagatgagttctattcacaattctaagtttacatgtcaaagttaacatgcccaaataatactttcctgtaatggaatgacaacccaaaaaatacactcaaaataataaacacaaaattcaaaaagtaacacaaaataatcctaccccagcagttgttccctaatctacaaagtcagaccaaaggatttctcaactttctttcaattctgactttttttaatagataatggaatcaaacactagtcacctttagctttatattacctaagaagtcacttattttttaacctctcagtaaagatactgagagttatttaaaaggtatcagctaagatattatctcctgatccaacaatcccacttctggctatttatccagaagatttgaaatccgtatgtcaaagagaagtctgcactctatgttcattgcagacaagtcacaataaccaagtgattcgatcaacctaagtgtccatccatggatgaatggataaagaaaatgtggcatatatatacaaaaaaatactattcagcctttaaaaaggaagaaattgtgtcatttgcaacaatatggatgatcgtggaggacattatggtaagtgaaataagccaagcacagaaagacaaataccacatgatctcacttatttgtgtaatctaaaacaattaaactcacagaagtagagagaagaatgatggttgctagaggccggggatgtgggaatagggagatgacaatcaaaagatacaaagcctcaattagatagaaggaatatgtttgactttttttagatctattacacaacatggtgaatacagctaataattaagcactgtatgtacatttcaatactgttgagagtacatttcaaatgttttcatcacaaaatatgtcaaatatttgaggtgatggatagattagctttatttaatcatcccacattatattcaaaaatcataatgccacttcgtacctcataagtatatacaactataatttgatatataataaaaaatttttaaaggtagtctcctaacaatcatatgaggattatcctaaaatgtcctttagtaactgtcatggactgaaaagtatcccatgaagagacaatgtctactcagaacatgtgaatacaaacttacttggaacatgggtctttgtaaacataattaagggtctccagacacaatcaccctagatcagggtgggccctacattcaaagacactgtccttaaaaggtaatgaaaagacagagggaaaggccgtgtgaacgcagaggcagagactggagtgaagattgctgtctgcaatacttagacaagatatgcccataagccaaagaactccaagaattgcagacagccacaagatattaggaaacagacatagaatggattcttccttagagcctccagaaggaaccaactctgctgacactttgattttagacttctggcctccagactgtgaggaaaattgttgtaagcacccaagtttgtggtcatttgttatggcagccctgggaagctaatacaatatgtatttcataaaggaaatcccccttttaaaggattataatcaacacaatttgtctttggccatcatacatttcatattaggaattagtgaaagagcttcatcatttctggattgtaaacaataaccaacaatttgatgcctagacagacatatatgagtctctactttatcatttactatctatgcatttctattttgacttagaattaaaattatatttactgaaatgttaaggaacttttcagtcaagaatatcacctgaccatttgtaaatatttgctaacacattgttattaggttggtacaaaagtaattgtggttttgccattactttcaatggcaaaaaccacaattacttttgcactaacctaatagttctctctgaagagaataaattagttctagtaatatgaagcatacccagttttaataaacttatacatacaaaacattcccaagctttgtgaggggccaacattacgagagcgatatgagatatctgaaaacaattttattttcccattattcaggcttttgaagcaggtcttaagctttcccagttctttgccacttaatttcttacatatgtttaaaatatatattaaaaaaactaatgtaatttgaggaccaccactgcacctaaaagaaattccatgttttccacctattcagttgttctttgtagaaatggtctaattattaagtccatttttacagttcaaaatatcactgatattaccacataaacctttgaatgtcctgactatttggccactgaaaagtcttgttcagaaagatgtaaaaagttatgaaattaacaattgcatagcaactcagttcacaaacaagtctggatgtgggaggcagagttatgttaagcctataaatgacataaggtaaaatgaagtaacgaaattccagcagtttctgaggaactataacaatgaacaagcatatgaaaaacattaaattccaaaaaattggctttgatttcaatgagtcagctatactccaaccagcaaatatataggctggaactaacaaatatttcagaattgcatatctttgaaaaactcttttccacacatagaaagtataatgtctattgtctgctagcaagtatttatgagcataagtgaatttccaaactaaaaacacagagactaaggtaaccaccaaaaacagaattccatgtttccaaactaaggaaagaaaagtcttaattttgctaggagacaggagatgaggaaaagaaaaaaagagagtaaatgaaaaaaagtagaatagttgaggaaaatgaagacaggcttcatgactactccgatcgccaataacaattccaccattaactactacaaaagcacaaaacagaaatcccagaaggatgtagggccaagtcaaacagaaaagcatactcaagtttttaaaggacatggaataagccaaaagaaactgaagaatttttctgaattctgcaaatggtcctttaataggtggaagtctgtcttccttcttttgtagctcagttttccaagcctcagttaacttttgtgcaatgacattccctgcacagaagacagcccagatgatatttgtttgccgaaacatgaagccacaaaatccaaggaaggctgaagttttatgatttccataaagacacatcaaatatgcaaaaagagtaaaaaacatagatcctgcttctgtataataaaggaagttaaaaaaataaagtgttggaaatactgctagtgttaatgttgacaagactctctggatacttgaggcagccttgtttctgggttgtaccttgtggaaaagcaaatatagtaaatagaagttgccaacactgaagagaagattaacaaatctgagcatcccaatggagcagacaacatgttcagaccatgcaaagatccaaatggcaggtttgaccactccaactgacaccaggtacaagccaggtaatgtagtaatcatgggatcccacggaaggcaaaggatgctgggagagcgcggatccggaaaacagcgggtcgctgtttcctggagtgacgggtttagataacggaccggatga

SEQ ID NO: 16835 - RNA, 7370 nt, Homo sapiens
  source 1..7370: mol_type = other RNA
tacgtagatatatatgtattttcttttccttgttagaaaaatactgtattgtcttttggtctgatggtgataggctgagataaaatttaattaacattaaattcatcaaaaatttatctcttaaaaaagcacaatatagagatattatattgtgacagaatttcttaccctagaaataatttttcaaatctcaaatattaaatattagtgttgactcatggatatatgttaaaaatatgtcctcaatctctatttttattataattttctcagttacacaagtttttgtatattggaaacgtcagttgtcaacattaaatacataaaaatgccctatataaaaaataattaacagctattcctagagtggtaaaatgtagcccaactaaaaaaaacaaagtatttgtaattagttgaaatgtcttttacctttaaattctttaacctgttattcgttgaaggttactgatttttcttattttaaatagaaataagaatattttcttattttaaataaaaagcaattattttgaaattatacccttaatagggtataaagtttctttaataagaaactttcctttaaagtgttataaccttttaatggttgaaagttatttgtttttcttattttaaataaacagtaattatgttgaaatcatatcctatcaaagaaacaacatgtttacaagtaaatacatgtataagcattaaatgctagcaggggtctccaatcttttggcttccctgggccacactggaagaaccatcttgggccacacataaaatacacgaacactaatgatagctgatgagctaaaaaataaaataaaataaaataaaataataaataaaataaaataaaataaaatcacaaaatatctcatcatgttttaagaaagcttacaaaatttgtgttggggccgcattcaaagccatcctgggctgcatgtggcctgtgggttgaacaagcttgcactaaggcaaataaaaattgttaacactgggtcagaaaattacacagaaaaatgtttaggatgactcttattatgaaacatgatttacttcctaaaattagccacggttatgtaggatgttttttctattcacttcactctatactaaaaacttcattcagtatatatttactcaatatttatcatatgacatacttataaatattatgagtatatggcaggaatgaatcctttttaaaataaggttatacacataccaatcagacactgactagagttaggacaaatactattctcatttgaaatgaggactaaagactaaaccacttgccttattgatcccagagccacaaccaaatataaaaatcttaactcccatgttaaatgtttttttctacaagcccacagttcctaagtcatatttcaatttccatttaaaaattttcaaatttatatcacaattcttacttgcttcactttttaatgaaattccaattacttcaaagataataaacgcttgctaacctaataaacacaaaatttatttcttcatgtgaataaatattttatttaaaagtgagtccaaaataacagtccactatttaggtggtataaataaaaatggtagatcccttcctctctcctctcttccaacaattctaaggaaaataatatcaagccaagtggcaattaagttcaaactagaaatacatttcattaagctacgtatttattagaaataaattacattaggctatttacacaagttattttatgactggctatgcacatttcagaaataactctaagaagacaaagaaaaggccagacagctaaaataatttatcttgccaaaatgagatgctaagtttaaactgagagatgctatctttccaaatcatttaaatacatagacgcagttcaaaagattcctgactatccattaatggaaaacataaacgttaacaaaattcacagcatacctgaatcttactcatgctacctaaagataacatatctctagaatttcacagaagatagaatcagttcaaaatgatgtattactgaacctataatgatttatggactagatatttttatgacacttttcaaaatagacatactcacagactttagtaatggtaactgtagggctccagatgccctcgagcagggcaatatttttttcataatcacctaattttaatcaattcagctaagtctaatgtttaaaaattcatgaaaaaatatctatctactcaataacttttgaaaacacaaatataactaagaatgtttctaaaagcaaggatctaaacacctaagaatggtcttctcagttgtttcaagtgaatgactttgagtttagtatcatttcttgaacgactaaaggcaaaatgatctgttgtgccaagttcttacataatcattttatctgttatctattttggaaaattcaccagcaaatggccatctttgaactgcctagaaaatttaacgaagacatttatcttaaattcgaaagtattgataagcattcctgttttaaaataataaatagttgaaaatagcaccttttaatacatggcattcttttcttaaaatgccaagtactatattttatgtattttataaaaaatgtggaagattaacctgtttctctctgaatgtagattttcaccaaaacatctcttaaacagcagggactcaacacttaaaaatgaactagaagagctgggcacagtggctcacgcctgtaatcccagcactttgggaggcgaggcaggtggattacctgaggtcaggagttcgagaccagcctggctaacacggtgaaaccccggctctactaaaaatagaaaaaattagccaggcttggtggtgggcgcctataatctcagctactcgggaggctgaggcaggagaactgcttgaacccaggaggtggaggtttcagtgagccaagatcgcgccattgcattccagcctgggggacaagagcgagacttctcctcaaagacaaaaacaaacaaaaaaagatatagaacagtgatccctccaaagagcagtcttctttaattacagggtagaatattttcctcaattttgccagactagatcagagtggaagcttctcctctcagaagtattcctaaatacaaaatccttgcattaatattatcagacaaaaagttactttccctaaattacacattcttttttcaattttgacttcccagatttagttctccactatagtaaattaatgacaaaagtataatttctttgagtgtcctctctcatctaatttttaagaagtctgggtaaaacacgtttttctacaatcactgttataactaatgccgatctattttctgagtactagagtacaaccaaaaaatggcctgcatttattactcaaattatacttgtaattttcacctgcacacaattttatatttgtaaatgtagactcatcacttaaaactcagagaagcaaaatttgacattgaggggaaagtaatttgttcacttatagctacttttaaagtttagaaacataaaattatgttaaaagatgagttctattcacaattctaagtttacatgtcaaagttaacatgcccaaataatactttcctgtaatggaatgacaacccaaaaaatacactcaaaataataaacacaaaattcaaaaagtaacacaaaataatcctaccccagcagttgttccctaatctacaaagtcagaccaaaggatttctcaactttctttcaattctgactttttttaatagataatggaatcaaacactagtcacctttagctttatattacctaagaagtcacttattttttaacctctcagtaaagatactgagagttatttaaaaggtatcagctaagatattatctcctgatccaacaatcccacttctggctatttatccagaagatttgaaatccgtatgtcaaagagaagtctgcactctatgttcattgcagacaagtcacaataaccaagtgattcgatcaacctaagtgtccatccatggatgaatggataaagaaaatgtggcatatatatacaaaaaaatactattcagcctttaaaaaggaagaaattgtgtcatttgcaacaatatggatgatcgtggaggacattatggtaagtgaaataagccaagcacagaaagacaaataccacatgatctcacttatttgtgtaatctaaaacaattaaactcacagaagtagagagaagaatgatggttgctagaggccggggatgtgggaatagggagatgacaatcaaaagatacaaagcctcaattagatagaaggaatatgtttgactttttttagatctattacacaacatggtgaatacagctaataattaagcactgtatgtacatttcaatactgttgagagtacatttcaaatgttttcatcacaaaatatgtcaaatatttgaggtgatggatagattagctttatttaatcatcccacattatattcaaaaatcataatgccacttcgtacctcataagtatatacaactataatttgatatataataaaaaatttttaaaggtagtctcctaacaatcatatgaggattatcctaaaatgtcctttagtaactgtcatggactgaaaagtatcccatgaagagacaatgtctactcagaacatgtgaatacaaacttacttggaacatgggtctttgtaaacataattaagggtctccagacacaatcaccctagatcagggtgggccctacattcaaagacactgtccttaaaaggtaatgaaaagacagagggaaaggccgtgtgaacgcagaggcagagactggagtgaagattgctgtctgcaatacttagacaagatatgcccataagccaaagaactccaagaattgcagacagccacaagatattaggaaacagacatagaatggattcttccttagagcctccagaaggaaccaactctgctgacactttgattttagacttctggcctccagactgtgaggaaaattgttgtaagcacccaagtttgtggtcatttgttatggcagccctgggaagctaatacaatatgtatttcataaaggaaatcccccttttaaaggattataatcaacacaatttgtctttggccatcatacatttcatattaggaattagtgaaagagcttcatcatttctggattgtaaacaataaccaacaatttgatgcctagacagacatatatgagtctctactttatcatttactatctatgcatttctattttgacttagaattaaaattatatttactgaaatgttaaggaacttttcagtcaagaatatcacctgaccatttgtaaatatttgctaacacattgttattaggttggtacaaaagtaattgtggttttgccattactttcaatggcaaaaaccacaattacttttgcactaacctaatagttctctctgaagagaataaattagttctagtaatatgaagcatacccagttttaataaacttatacatacaaaacattcccaagctttgtgaggggccaacattacgagagcgatatgagatatctgaaaacaattttattttcccattattcaggcttttgaagcaggtcttaagctttcccagttctttgccacttaatttcttacatatgtttaaaatatatattaaaaaaactaatgtaatttgaggaccaccactgcacctaaaagaaattccatgttttccacctattcagttgttctttgtagaaatggtctaattattaagtccatttttacagttcaaaatatcactgatattaccacataaacctttgaatgtcctgactatttggccactgaaaagtcttgttcagaaagatgtaaaaagttatgaaattaacaattgcatagcaactcagttcacaaacaagtctggatgtgggaggcagagttatgttaagcctataaatgacataaggtaaaatgaagtaacgaaattccagcagtttctgaggaactataacaatgaacaagcatatgaaaaacattaaattccaaaaaattggctttgatttcaatgagtcagctatactccaaccagcaaatatataggctggaactaacaaatatttcagaattgcatatctttgaaaaactcttttccacacatagaaagtataatgtctattgtctgctagcaagtatttatgagcataagtgaatttccaaactaaaaacacagagactaaggtaaccaccaaaaacagaattccatgtttccaaactaaggaaagaaaagtcttaattttgctaggagacaggagatgaggaaaagaaaaaaagagagtaaatgaaaaaaagtagaatagttgaggaaaatgaagacaggcttcatgactactccgatcgccaataacaattccaccattaactactacaaaagcacaaaacagaaatcccagaaggatgtagggccaagtcaaacagaaaagcatactcaagtttttaaaggacatggaataagccaaaagaaactgaagaatttttctgaattctgcaaatggtcctttaataggtggaagtctgtcttccttcttttgtagctcagttttccaagcctcagttaacttttgtgcaatgacattccctgcacagaagacagcccagatgatatttgtttgccgaaacatgaagccacaaaatccaaggaaggctgaagttttatgatttccataaagacacatcaaatatgcaaaaagagtaaaaaacatagatcctgcttctgtataataaaggaagttaaaaaaataaagtgttggaaatactgctagtgttaatgttgacaagactctctggatacttgaggcagccttgtttctgggttgtaccttgtggaaaagcaaatatagtaaatagaagttgccaacactgaagagaagattaacaaatctgagcatcccaatggagcagacaacatgttcagaccatgcaaagatccaaatggcaggtttgaccactccaactgacaccaggtacaagccaggtaatgtagtaatcatgggatcccactgggaaagggagaaatggccctcacagtagcgctgcgcctgaggcaggtggaagatctcgtccatgtagggctctcgcagcgcccggctgaaggcggagaagaggaggcaggacactaaaaaggtacagctcaaggcggccgagaaacagtaaccctctagctgcgccattcctgctcccacagccactgcccaagaacccactcctggaaaattctgagcccggaaacccgagctggaaacttgggctcgaaatgggcgcgctagacaggactagccagacggggccac

SEQ ID NO: 16836 - RNA, 3618 nt, Homo sapiens
  source 1..3618: mol_type = other RNA
tacgtagatatatatgtattttcttttccttgttagaaaaatactgtattgtcttttggtctgatggtgataggctgagataaaatttaattaacattaaattcatcaaaaatttatctcttaaaaaagcacaatatagagatattatattgtgacagaatttcttaccctagaaataatttttcaaatctcaaatattaaatattagtgttgactcatggatatatgttaaaaatatgtcctcaatctctatttttattataattttctcagttacacaagtttttgtatattggaaacgtcagttgtcaacattaaatacataaaaatgccctatataaaaaataattaacagctattcctagagtggtaaaatgtagcccaactaaaaaaaacaaagtatttgtaattagttgaaatgtcttttacctttaaattctttaacctgttattcgttgaaggttactgatttttcttattttaaatagaaataagaatattttcttattttaaataaaaagcaattattttgaaattatacccttaatagggtataaagtttctttaataagaaactttcctttaaagtgttataaccttttaatggttgaaagttatttgtttttcttattttaaataaacagtaattatgttgaaatcatatcctatcaaagaaacaacatgtttacaagtaaatacatgtataagcattaaatgctagcaggggtctccaatcttttggcttccctgggccacactggaagaaccatcttgggccacacataaaatacacgaacactaatgatagctgatgagctaaaaaataaaataaaataaaataaaataataaataaaataaaataaaataaaatcacaaaatatctcatcatgttttaagaaagcttacaaaatttgtgttggggccgcattcaaagccatcctgggctgcatgtggcctgtgggttgaacaagcttgcactaaggcaaataaaaattgttaacactgggtcagaaaattacacagaaaaatgtttaggatgactcttattatgaaacatgatttacttcctaaaattagccacggttatgtaggatgttttttctattcacttcactctatactaaaaacttcattcagtatatatttactcaatatttatcatatgacatacttataaatattatgagtatatggcaggaatgaatcctttttaaaataaggttatacacataccaatcagacactgactagagttaggacaaatactattctcatttgaaatgaggactaaagactaaaccacttgccttattgatcccagagccacaaccaaatataaaaatcttaactcccatgttaaatgtttttttctacaagcccacagttcctaagtcatatttcaatttccatttaaaaattttcaaatttatatcacaattcttacttgcttcactttttaatgaaattccaattacttcaaagataataaacgcttgctaacctaataaacacaaaatttatttcttcatgtgaataaatattttatttaaaagtgagtccaaaataacagtccactatttaggtggtataaataaaaatggtagatcccttcctctctcctctcttccaacaattctaaggaaaataatatcaagccaagtggcaattaagttcaaactagaaatacatttcattaagctacgtatttattagaaataaattacattaggctatttacacaagttattttatgactggctatgcacatttcagaaataactctaagaagacaaagaaaaggccagacagctaaaataatttatcttgccaaaatgagatgctaagtttaaactgagagatgctatctttccaaatcatttaaatacatagacgcagttcaaaagattcctgactatccattaatggaaaacataaacgttaacaaaattcacagcatacctgaatcttactcatgctacctaaagataacatatctctagaatttcacagaagatagaatcagttcaaaatgatgtattactgaacctataatgatttatggactagatatttttatgacacttttcaaaatagacatactcacagactttagtaatggtaactgtagggctccagatgccctcgagcagggcaatatttttttcataatcacctaattttaatcaattcagctaagtctaatgtttaaaaattcatgaaaaaatatctatctactcaataacttttgaaaacacaaatataactaagaatgtttctaaaagcaaggatctaaacacctaagaatggtcttctcagttgtttcaagtgaatgactttgagtttagtatcatttcttgaacgactaaaggcaaaatgatctgttgtgccaagttcttacataatcattttatctgttatctattttggaaaattcaccagcaaatggccatctttgaactgcctagaaaatttaacgaagacatttatcttaaattcgaaagtattgataagcattcctgttttaaaataataaatagttgaaaatagcaccttttaatacatggcattcttttcttaaaatgccaagtactatattttatgtattttataaaaaatgtggaagattaacctgtttctctctgaatgtagattttcaccaaaacatctcttaaacagcagggactcaacacttaaaaatgaactagaagagctgggcacagtggctcacgcctgtaatcccagcactttgggaggcgaggcaggtggattacctgaggtcaggagttcgagaccagcctggctaacacggtgaaaccccggctctactaaaaatagaaaaaattagccaggcttggtggtgggcgcctataatctcagctactcgggaggctgaggcaggagaactgcttgaacccaggaggtggaggtttcagtgagccaagatcgcgccattgcattccagcctgggggacaagagcgagacttctcctcaaagacaaaaacaaacaaaaaaagatatagaacagtgatccctccaaagagcagtcttctttaattacagggtagaatattttcctcaattttgccagactagatcagagtggaagcttctcctctcagaagtattccttgtttctgggttgtaccttgtggaaaagcaaatatagtaaatagaagttgccaacactgaagagaagattaacaaatctgagcatcccaatggagcagacaacatgttcagaccatgcaaagatccaaatggcaggtttgaccactccaactgacaccaggtacaagccaggtaatgtagtaatcatgggatcccactgggaaagggagaaatggccctcacagtagcgctgcgcctgaggcaggtggaagatctcgtccatgtagggctctcgcagcgcccggctgaaggcggagaagaggaggcaggacactaaaaaggtacagctcaaggcggccgagaaacagtaaccctctagctgcgccattcctgctcccacagccactgcccaagaacccactcctggaaaattctgagcccggaaacccgagctggaaacttgggctcgaaatgggcgcgctagacaggactagccagacggggccac

SEQ ID NO: 16837 - RNA, 2064 nt, Homo sapiens
  source 1..2064: mol_type = other RNA
tacgtagatatatatgtatttttaaatatagaaaaactccaccaatagtagaaacaaagtatgtttaatggttgctttggaaaggggaagtgggcacctcatgccagggagatttaaaaatgagacttttcaagcaagcactgcctatagcatagtctcatattttgaaaatttaaacctaattttaattatatataaagaactattttaaaaaatcacacccacaagtaaaaaactggtaatctgtttacaaagtgcagcgtcagtacagcaaactcatctcaacaaaagattatgtgtggtttctcgggctttaaaactcccctggtttccatttaaatgctttaacattgagtcatcctgcatacatgaaaagcctgtgtaatgaagcctgggtcctttaacacctgctattaattaattccaacataagtgagtatgagacctgggaagtaaattgtcatcatctgattgatgaggtacagattatctgaataaaatttctgacctggttatgagtcagtaatcccaacacaaactactgctttgtaatgaattctgtatgctttgcatgtccttcaataactgaagattttttctccttttttctccaggtctcagtttcataaaatctttcttatttgtggtccctgtgattccagaacggctgctgctgtttctttcttcatcaagagtctttttggtagcttttaattccttcttctgcttctctaacttctgtttctccagctgggcttggtattttcgaactttagttatttggttggcttttgcttccatccttcccactaatgcctccaattcacactccaacttgtctttcagttcaacggttggcgactcctggataagttttgcaagctgctggtgatcaaagctcatttgcccaaattcatcctgtaaagtctgtaagacttctgacaactcctcattaataccgttggaggagggaggtgttactgacaacttcttacttttaccacctcgtgaagatacttgctttgccaaaggaatactgttgatgactcgatcattgcacaaagctttactgtgttgcttcattagatgcaagacaagctgaacattggctaccacggcatggctagggcttgtggactcagctgccttagcttgcatgcgtttcctttcctgttcttcttcatggagttttgcttccaactcttgcatttttttttctgcaagggcctgcattgtggtaagtttgttatactcctgttcaagaagatccaatttttcaagttggctctgaacatgtgtttgatcatgttgtcgttctctttctagggaaacttgtttctctaagacagatgtcctctccatttcggcatgctttatcatatttcgcatgtattccaattgtttttctaatagattgcatttattttctgcagctaacaactgagatgtcagttcttgattgtgctttgattcctcattctttgaattctccctttcttgtatctgttcatccagtactttcttatattcaattgtttctctagacaaggttttcacactttcttctgcctgaatcctctcaagttccaagcgtcgaatcttatcttgaagattcttaagagcagaaaatatggctctgctgttgctttctggataggcaagtgtaggcttacttggggagcgtcgtagatcactattaaggaaaggcttatccgaaggatatactacatatggagatgaagaatgccgaaccatgcttccattagaccttgatggctcagcaaagctgttcgacaagtgagaaccagaagccgcagagacagacgccgccgccatctttcagcctgcccagggggtctccgcacttcgggggcggtctaggttctcgtgctcttctccaagactcgggagccgcccaccagcggggaccctaggctgaacccctgatggaaaagggcaagggtgctggtgctgggcttggaaacccctgcaacacaccccctcagggccgcctacgctcacagcttacacagaaagggcaacacgtcctaacggacgtctttc

SEQ ID NO: 16838 - RNA, 1947 nt, Homo sapiens
  source 1..1947: mol_type = other RNA
tacgtagatatatatgtatttttaaatatagaaaaactccaccaatagtagaaacaaagtatgtttaatggttgctttggaaaggggaagtgggcacctcatgccagggagatttaaaaatgagacttttcaagcaagcactgcctatagcatagtctcatattttgaaaatttaaacctaattttaattatatataaagaactattttaaaaaatcacacccacaagtaaaaaactggtaatctgtttacaaagtgcagcgtcagtacagcaaactcatctcaacaaaagattatgtgtggtttctcgggctttaaaactcccctggtttccatttaaatgctttaacattgagtcatcctgcatacatgaaaagcctgtgtaatgaagcctgggtcctttaacacctgctattaattaattccaacataagtgagtatgagacctgggaagtaaattgtcatcatctgattgatgaggtacagattatctgaataaaatttctgacctggttatgagtcagtaatcccaacacaaactactgctttgtaatgaattctgtatgctttgcatgtccttcaataactgaagattttttctccttttttctccaggtctcagtttcataaaatctttcttatttgtggtccctgtgattccagaacggctgctgctgtttctttcttcatcaagagtctttttggtagcttttaattccttcttctgcttctctaacttctgtttctccagctgggcttggtattttcgaactttagttatttggttggcttttgcttccatccttcccactaatgcctccaattcacactccaacttgtctttcagttcaacggttggcgactcctggataagttttgcaagctgctggtgatcaaagctcatttgcccaaattcatcctgtaaagtctgtaagacttctgacaactcctcattaataccgttggaggagggaggtgttactgacaacttcttacttttaccacctcgtgaagatacttgctttgccaaaggaatactgttgatgactcgatcattgcacaaagctttactgtgttgcttcattagatgcaagacaagctgaacattggctaccacggcatggctagggcttgtggactcagctgccttagcttgcatgcgtttcctttcctgttcttcttcatggagttttgcttccaactcttgcatttttttttgtttctctaagacagatgtcctctccatttcggcatgctttatcatatttcgcatgtattccaattgtttttctaatagattgcatttattttctgcagctaacaactgagatgtcagttcttgattgtgctttgattcctcattctttgaattctccctttcttgtatctgttcatccagtactttcttatattcaattgtttctctagacaaggttttcacactttcttctgcctgaatcctctcaagttccaagcgtcgaatcttatcttgaagattcttaagagcagaaaatatggctctgctgttgctttctggataggcaagtgtaggcttacttggggagcgtcgtagatcactattaaggaaaggcttatccgaaggatatactacatatggagatgaagaatgccgaaccatgcttccattagaccttgatggctcagcaaagctgttcgacaagtgagaaccagaagccgcagagacagacgccgccgccatctttcagcctgcccagggggtctccgcacttcgggggcggtctaggttctcgtgctcttctccaagactcgggagccgcccaccagcggggaccctaggctgaacccctgatggaaaagggcaagggtgctggtgctgggcttggaaacccctgcaacacaccccctcagggccgcctacgctcacagcttacacagaaagggcaacacgtcctaacggacgtctttc

SEQ ID NO: 16839 - RNA, 2663 nt, Homo sapiens
  source 1..2663: mol_type = other RNA
tacgtagatatatatgtatttttaaatatagaaaaactccaccaatagtagaaacaaagtatgtttaatggttgctttggaaaggggaagtgggcacctcatgccagggagatttaaaaatgagacttttcaagcaagcactgcctatagcatagtctcatattttgaaaatttaaacctaattttaattatatataaagaactattttaaaaaatcacacccacaagtaaaaaactggtaatctgtttacaaagtgcagcgtcagtacagcaaactcatctcaacaaaagattatgtgtggtttctcgggctttaaaactcccctggtttccatttaaatgctttaacattgagtcatcctgcatacatgaaaagcctgtgtaatgaagcctgggtcctttaacacctgctattaattaattccaacataagtgagtatgagacctgggaagtaaattgtcatcatctgattgatgaggtacagattatctgaataaaatttctgacctggttatgagtcagtaatcccaacacaaactactgctttgtaatgaattctgtatgctttgcatgtccttcaataactgaagattttttctccttttttctccaggtctcagtttcataaaatctttcttatttgtggtccctgtgattccagaacggctgctgctgtttctttcttcatcaagagtctttttggtagcttttaattccttcttctgcttctctaacttctgtttctccagctgggcttggtattttcgaactttagttatttggttggcttttgcttccatccttcccactaatgcctccaattcacactccaacttgtctttcagttcaacggttggcgactcctggataagttttgcaagctgctggtgatcaaagctcatttgcccaaattcatcctgtaaagtctgtaagacttctgacaactcctcattaataccgttggaggagggaggtgttactgacaacttcttacttttaccacctcgtgaagatacttgctttgccaaaggaatactgttgatgactcgatcattgcacaaagctttactgtgttgcttcattagatgcaagacaagctgaacattggctaccacggcatggctagggcttgtggacttcccagctacaaatggcatatcacccaagcataatctataatgtggttgtgcaccaaaatagttcctagaacttttcttatctatagttggcattatgatcacaagccagctcctaatagtacttgttagcatatatcctagcctaggaaaggctggggggaaaaaagcacttgacaaaacaacagttacattctaagtagaaaatcagtatacatatacacaaaacattgtaagagcacaagataatgcagtactaataatgctaattttgtatggtgttctgtagttccaaaatgcttatatattttctcactatcaggataaaaatttaggagtaggtattacttatctccaccttctgaatgaagaaattgagaatgaaagatttactctctcaaggttgtagtacaccacacagtttatgggtgttttgacataaactataccaagtaatcagcattttgcctgatttggttctgtcttcacaccttttctggtggttttgacttcttttttttaattcttcttgcattgggaacacacggagttgccttatcttcaaagataagtctatttgtttctagaccagtctgcaactcagctgccttagcttgcatgcgtttcctttcctgttcttcttcatggagttttgcttccaactcttgcatttttttttctgcaagggcctgcattgtggtaagtttgttatactcctgttcaagaagatccaatttttcaagttggctctgaacatgtgtttgatcatgttgtcgttctctttctagggaaacttgtttctctaagacagatgtcctctccatttcggcatgctttatcatatttcgcatgtattccaattgtttttctaatagattgcatttattttctgcagctaacaactgagatgtcagttcttgattgtgctttgattcctcattctttgaattctccctttcttgtatctgttcatccagtactttcttatattcaattgtttctctagacaaggttttcacactttcttctgcctgaatcctctcaagttccaagcgtcgaatcttatcttgaagattcttaagagcagaaaatatggctctgctgttgctttctggataggcaagtgtaggcttacttggggagcgtcgtagatcactattaaggaaaggcttatccgaaggatatactacatatggagatgaagaatgccgaaccatgcttccattagaccttgatggctcagcaaagctgttcgacaagtgagaaccagaagccgcagagacagacgccgccgccatctttcagcctgcccagggggtctccgcacttcgggggcggtctaggttctcgtgctcttctccaagactcgggagccgcccaccagcggggaccctaggctgaacccctgatggaaaagggcaagggtgctggtgctgggcttggaaacccctgcaacacaccccctcagggccgcctacgctcacagcttacacagaaagggcaacacgtcctaacggacgtctttc

SEQ ID NO: 16840 - RNA, 3450 nt, Homo sapiens
  source 1..3450: mol_type = other RNA
tacgtagatatatatgtatttttaaatatagaaaaactccaccaatagtagaaacaaagtatgtttaatggttgctttggaaaggggaagtgggcacctcatgccagggagatttaaaaatgagacttttcaagcaagcactgcctatagcatagtctcatattttgaaaatttaaacctaattttaattatatataaagaactattttaaaaaatcacacccacaagtaaaaaactggtaatctgtttacaaagtgcagcgtcagtacagcaaactcatctcaacaaaagattatgtgtggtttctcgggctttaaaactcccctggtttccatttaaatgctttaacattgagtcatcctgcatacatgaaaagcctgtgtaatgaagcctgggtcctttaacacctgctattaattaattccaacataagtgagtatgagacctgggaagtaaattgtcatcatctgattgatgaggtacagattatctgaataaaatttctgacctggttatgagtcagtaatcccaacacaaactactgctttgtaatgaattctgtatgctttgcatgtccttcaataactgaagattttttctccttttttctccaggtctcagtttcataaaatctttcttatttgtggtccctgtgattccagaacggctgctgctgtttctttcttcatcaagagtctttttggtagcttttaattccttcttctgcttctctaacttctgtttctccagctgggcttggtattttcgaactttagttatttggttggcttttgcttccatccttcccactaatgcctccaattcacactccaacttgtctttcagttcaacggttggcgactcctggataagttttgcaagctgctggtgatcaaagctcatttgcccaaattcatcctgtaaagtctgtaagacttctgacaactcctcattaataccgttggaggagggaggtgttactgacaacttcttacttttaccacctcgtgaagatacttgctttgccaaaggaatactgttgatgactcgatcattgcacaaagctttactgtgttgcttcattagatgcaagacaagctgaacattggctaccacggcatggctagggcttgtggacttcccagctacaaatggcatatcacccaagcataatctataatgtggttgtgcaccaaaatagttcctagaacttttcttttctggtggttttgacttcttttttttaattcttcttgcattgggaacacacggagttgccttatcttcaaagataagtctatttgtttctagaccagtctgcaactcagctgccttagcttgcatgcgtttcctttcctgttcttcttcatggagttttgcttccaactcttgcatttttttttctgcaagggcctgcattgtggtaagtttgttatactcctgttcaagaagatccaatttttcaagttggctctgaacatgtgtttgatcatgttgtcgttctctttctagggaaacttgtttctctaagacagatgtcctctccatttcggcatgctttatcatatttcgcatgtattccaattgtttttctaatagattgcatttattttctgcagctaacaactgagatgtcagttcttgattgtgctttgattcctcattctttgaattctccctttcttgtatctgttcatccagtactttcttatattcaattgtttctctagacaaggttttcacactttcttctgcctgaatcctctcaagttccaagcgtcgaatcttatcttgaagattcttaagagcagaaaatatggctctgctgttgctttctggataggcaagtgtaggcttacttggggagcgtcgtagatcactattaaggaaaggcttatccgaaggatatactacatatggagatgaagaatgccgaaccatgcttccattagaccttgatggctcagcaaagctgttatcaattctggtcaacattgtacttcatttccctagtctgcacacaatgataagaggtgcacaaatcagaaaataggataccatttcacacacacagcaaaaatttacaagtgggacgataccatccatttaagaggacataaaataaagagggttgttggtataatcacttggtaaaacaatttagtatgaccgagtaaagctgaagacgcacatactctgtgaaccagataattcattcagttatatttgctgaacgattttctctctcttctttcttgaaaatgatacgggttgagtcacagtacatattccatgacccactactgagctgtaatccagagcccagcctctggtctggaaaaaaaaaagaaaaatcactgccctagagttgccccttgcaaactttttctctcaggacccctttacactctaaaagatctagtgaaaagaatggcactattttacatttctgcagatctctttaatgtttgctttaaaaaaagaatgctggattctcttatctagttctgcattcgctctgttggatatgttattttgtttgacttattaaagatctagtctaccacaaacgtggtcattacagaaggatcttgtagactctgagagggtcttggagatctccaagggttgtgagaccatacttcgagaactgcactctagagaaacatttgccatgtacagcatataacaatgaatacaagattgtttctaatatctggcaaacaaatgaacagcaaaacccattaaatccaaagcccattaagatactgtcatttactagctagagaactttgactcaacctctctgtgcctcattttgctcatttgaaaaaggaaatattaatgccaatctcagaaggttattgtgaggattaaatgagttaatgcatgaaaagggtctttaaggattatgccttgccaggtagtcctatataaataccatacattataatcttaaaatacgtggtagtgggtgggtgtgggaaggagaaagaagacacagaggaacatgaaggtattcattttattattctcaaaaagtaaatcttatatttaatattataaaatgtatgatagccataaaacatttttaagggaaattaatatggagctactgtgcagcttggtcgaaggaccaaaagtcagagggacaaatcaagagattaggtcattaatcaccaaggttattgtgaaaatattacaaggctgacatgaaagacattcttgtgtatttcaacacaatgctgcccatacctccatatggaattaatttcattatgcccaatcatagttgctttcctgccttttccaccagtcgaagtttatcaattccagagcaatcactcaataaacgttacctagaacctaactgaaacctatcgccctacttccatgctgttcacatttgagatttacatggtcactgcttcccaaagacggttatttatg

SEQ ID NO: 16841 - RNA, 2267 nt, Homo sapiens
  source 1..2267: mol_type = other RNA
tacgtagatatatatgtatttttaaatatagaaaaactccaccaatagtagaaacaaagtatgtttaatggttgctttggaaaggggaagtgggcacctcatgccagggagatttaaaaatgagacttttcaagcaagcactgcctatagcatagtctcatattttgaaaatttaaacctaattttaattatatataaagaactattttaaaaaatcacacccacaagtaaaaaactggtaatctgtttacaaagtgcagcgtcagtacagcaaactcatctcaacaaaagattatgtgtggtttctcgggctttaaaactcccctggtttccatttaaatgctttaacattgagtcatcctgcatacatgaaaagcctgtgtaatgaagcctgggtcctttaacacctgctattaattaattccaacataagtgagtatgagacctgggaagtaaattgtcatcatctgattgatgaggtacagattatctgaataaaatttctgacctggttatgagtcagtaatcccaacacaaactactgctttgtaatgaattctgtatgctttgcatgtccttcaataactgaagattttttctccttttttctccaggtctcagtttcataaaatctttcttatttgtggtccctgtgattccagaacggctgctgctgtttctttcttcatcaagagtctttttggtagcttttaattccttcttctgcttctctaacttctgtttctccagctgggcttggtattttcgaactttagttatttggttggcttttgcttccatccttcccactaatgcctccaattcacactccaacttgtctttcagttcaacggttggcgactcctggataagttttgcaagctgctggtgatcaaagctcatttgcccaaattcatcctgtaaagtctgtaagacttctgacaactcctcattaataccgttggaggagggaggtgttactgacaacttcttacttttaccacctcgtgaagatacttgctttgccaaaggaatactgttgatgactcgatcattgcacaaagctttactgtgttgcttcattagatgcaagacaagctgaacattggctaccacggcatggctagggcttgtggacttcccagctacaaatggcatatcacccaagcataatctataatgtggttgtgcaccaaaatagttcctagaacttttcttttctggtggttttgacttcttttttttaattcttcttgcattgggaacacacggagttgccttatcttcaaagataagtctatttgtttctagaccagtctgcaactcagctgccttagcttgcatgcgtttcctttcctgttcttcttcatggagttttgcttccaactcttgcatttttttttctgcaagggcctgcattgtggtaagtttgttatactcctgttcaagaagatccaatttttcaagttggctctgaacatgtgtttgatcatgttgtcgttctctttctagggaaacttgtttctctaagacagatgtcctctccatttcggcatgctttatcatatttcgcatgtattccaattgtttttctaatagattgcatttattttctgcagctaacaactgagatgtcagttcttgattgtgctttgattcctcattctttgaattctccctttcttgtatctgttcatccagtactttcttatattcaattgtttctctagacaaggttttcacactttcttctgcctgaatcctctcaagttccaagcgtcgaatcttatcttgaagattcttaagagcagaaaatatggctctgctgttgctttctggataggcaagtgtaggcttacttggggagcgtcgtagatcactattaaggaaaggcttatccgaaggatatactacatatggagatgaagaatgccgaaccatgcttccattagaccttgatggctcagcaaagctgttatcaattctggtcaacattgtacttcatttccctagtctgcacacgacaagtgagaaccagaagccgcagagacagacgccgccgccatctttcagcctgcccagggggtctccgcacttcgggggcggtctaggttctcgtgctcttctccaagactcgggagccgcccaccagcggggaccctaggctgaacccctgatggaaaagggcaagggtgctggtgctgggcttggaaacccctgcaacacaccccctcagggccgcctacgctcacagcttacacagaaag

SEQ ID NO: 16842 - RNA, 2536 nt, Homo sapiens
  source 1..2536: mol_type = other RNA
tacgtagatatatatgtatttttaaatatagaaaaactccaccaatagtagaaacaaagtatgtttaatggttgctttggaaaggggaagtgggcacctcatgccagggagatttaaaaatgagacttttcaagcaagcactgcctatagcatagtctcatattttgaaaatttaaacctaattttaattatatataaagaactattttaaaaaatcacacccacaagtaaaaaactggtaatctgtttacaaagtgcagcgtcagtacagcaaactcatctcaacaaaagattatgtgtggtttctcgggctttaaaactcccctggtttccatttaaatgctttaacattgagtcatcctgcatacatgaaaagcctgtgtaatgaagcctgggtcctttaacacctgctattaattaattccaacataagtgagtatgagacctgggaagtaaattgtcatcatctgattgatgaggtacagattatctgaataaaatttctgacctggttatgagtcagtaatcccaacacaaactactgctttgtaatgaattctgtatgctttgcatgtccttcaataactgaagattttttctccttttttctccaggtctcagtttcataaaatctttcttatttgtggtccctgtgattccagaacggctgctgctgtttctttcttcatcaagagtctttttggtagcttttaattccttcttctgcttctctaacttctgtttctccagctgggcttggtattttcgaactttagttatttggttggcttttgcttccatccttcccactaatgcctccaattcacactccaacttgtctttcagttcaacggttggcgactcctggataagttttgcaagctgctggtgatcaaagctcatttgcccaaattcatcctgtaaagtctgtaagacttctgacaactcctcattaataccgttggaggagggaggtgttactgacaacttcttacttttaccacctcgtgaagatacttgctttgccaaaggaatactgttgatgactcgatcattgcacaaagctttactgtgttgcttcattagatgcaagacaagctgaacattggctaccacggcatggctagggcttgtggacttcccagctacaaatggcatatcacccaagcataatctataatgtggttgtgcaccaaaatagttcctagaacttttcttttctggtggttttgacttcttttttttaattcttcttgcattgggaacacacggagttgccttatcttcaaagataagtctatttgtttctagaccagtctgcaactcagctgccttagcttgcatgcgtttcctttcctgttcttcttcatggagttttgcttccaactcttgcatttttttttctgcaagggcctgcattgtggtaagtttgttatactcctgttcaagaagatccaatttttcaagttggctctgaacatgtgtttgatcatgttgtcgttctctttctagggaaacttgtttctctaagacagatgtcctctccatttcggcatgctttatcatatttcgcatgtattccaattgtttttctaatagattgcatttattttctgcagctaacaactgagatgtcagttcttgattgtgctttgattcctcattctttgaattctccctttcttgtatctgttcatccagtactttcttatattcaattgtttctctagacaaggttttcacactttcttctgcctgaatcctctcaagttccaagcgtcgaatcttatcttgaagattcttaagagcagaaaatatggctctgctgttgctttctggataggcaagtgtaggcttacttggggagcgtcgtagatcactattaaggaaaggcttatccgaaggatatactacatatggagatgaagaatgccgaaccatgcttccattagaccttgatggctcagcaaagctgttcaatgataagaggtgcacaaatcagaaaataggataccatttcacacacacagcaaaaatttacaagtgggacgataccatccatttaagaggacataaaataaagagggttgttggtataatcacttggtaaaacaatttagtatgaccgagtaaagctgaagacgcacatactctgtgaaccagataattcattcagttatatttgctgaacgattttctctctcttctttcttgaaaatgatacgggttgagtcacagtacatattccatgacccactactgagctgtaatccagagcccagcctctggtcgacaagtgagaaccagaagccgcagagacagacgccgccgccatctttcagcctgcccagggggtctccgcacttcgggggcggtctaggttctcgtgctcttctccaagactcgggagccgcccaccagcggggaccctaggctgaacccctgatggaaaagggcaagggtgctggtgctgggcttggaaacccctgcaacacaccccctcagggccgcctacgctcacagcttacacagaaag

SEQ ID NO: 16843 - RNA, 2223 nt, Homo sapiens
  source 1..2223: mol_type = other RNA
tacgtagatatatatgtatttttaaatatagaaaaactccaccaatagtagaaacaaagtatgtttaatggttgctttggaaaggggaagtgggcacctcatgccagggagatttaaaaatgagacttttcaagcaagcactgcctatagcatagtctcatattttgaaaatttaaacctaattttaattatatataaagaactattttaaaaaatcacacccacaagtaaaaaactggtaatctgtttacaaagtgcagcgtcagtacagcaaactcatctcaacaaaagattatgtgtggtttctcgggctttaaaactcccctggtttccatttaaatgctttaacattgagtcatcctgcatacatgaaaagcctgtgtaatgaagcctgggtcctttaacacctgctattaattaattccaacataagtgagtatgagacctgggaagtaaattgtcatcatctgattgatgaggtacagattatctgaataaaatttctgacctggttatgagtcagtaatcccaacacaaactactgctttgtaatgaattctgtatgctttgcatgtccttcaataactgaagattttttctccttttttctccaggtctcagtttcataaaatctttcttatttgtggtccctgtgattccagaacggctgctgctgtttctttcttcatcaagagtctttttggtagcttttaattccttcttctgcttctctaacttctgtttctccagctgggcttggtattttcgaactttagttatttggttggcttttgcttccatccttcccactaatgcctccaattcacactccaacttgtctttcagttcaacggttggcgactcctggataagttttgcaagctgctggtgatcaaagctcatttgcccaaattcatcctgtaaagtctgtaagacttctgacaactcctcattaataccgttggaggagggaggtgttactgacaacttcttacttttaccacctcgtgaagatacttgctttgccaaaggaatactgttgatgactcgatcattgcacaaagctttactgtgttgcttcattagatgcaagacaagctgaacattggctaccacggcatggctagggcttgtggacttcccagctacaaatggcatatcacccaagcataatctataatgtggttgtgcaccaaaatagttcctagaacttttcttttctggtggttttgacttcttttttttaattcttcttgcattgggaacacacggagttgccttatcttcaaagataagtctatttgtttctagaccagtctgcaactcagctgccttagcttgcatgcgtttcctttcctgttcttcttcatggagttttgcttccaactcttgcatttttttttctgcaagggcctgcattgtggtaagtttgttatactcctgttcaagaagatccaatttttcaagttggctctgaacatgtgtttgatcatgttgtcgttctctttctagggaaacttgtttctctaagacagatgtcctctccatttcggcatgctttatcatatttcgcatgtattccaattgtttttctaatagattgcatttattttctgcagctaacaactgagatgtcagttcttgattgtgctttgattcctcattctttgaattctccctttcttgtatctgttcatccagtactttcttatattcaattgtttctctagacaaggttttcacactttcttctgcctgaatcctctcaagttccaagcgtcgaatcttatcttgaagattcttaagagcagaaaatatggctctgctgttgctttctggataggcaagtgtaggcttacttggggagcgtcgtagatcactattaaggaaaggcttatccgaaggatatactacatatggagatgaagaatgccgaaccatgcttccattagaccttgatggctcagcaaagctgttcgacaagtgagaaccagaagccgcagagacagacgccgccgccatctttcagcctgcccagggggtctccgcacttcgggggcggtctaggttctcgtgctcttctccaagactcgggagccgcccaccagcggggaccctaggctgaacccctgatggaaaagggcaagggtgctggtgctgggcttggaaacccctgcaacacaccccctcagggccgcctacgctcacagcttacacagaaag

SEQ ID NO: 16844 - RNA, 2173 nt, Homo sapiens
  source 1..2173: mol_type = other RNA
tacgtagatatatatgtatttttaaatatagaaaaactccaccaatagtagaaacaaagtatgtttaatggttgctttggaaaggggaagtgggcacctcatgccagggagatttaaaaatgagacttttcaagcaagcactgcctatagcatagtctcatattttgaaaatttaaacctaattttaattatatataaagaactattttaaaaaatcacacccacaagtaaaaaactggtaatctgtttacaaagtgcagcgtcagtacagcaaactcatctcaacaaaagattatgtgtggtttctcgggctttaaaactcccctggtttccatttaaatgctttaacattgagtcatcctgcatacatgaaaagcctgtgtaatgaagcctgggtcctttaacacctgctattaattaattccaacataagtgagtatgagacctgggaagtaaattgtcatcatctgattgatgaggtacagattatctgaataaaatttctgacctggttatgagtcagtaatcccaacacaaactactgctttgtaatgaattctgtatgctttgcatgtccttcaataactgaagattttttctccttttttctccaggtctcagtttcataaaatctttcttatttgtggtccctgtgattccagaacggctgctgctgtttctttcttcatcaagagtctttttggtagcttttaattccttcttctgcttctctaacttctgtttctccagctgggcttggtattttcgaactttagttatttggttggcttttgcttccatccttcccactaatgcctccaattcacactccaacttgtctttcagttcaacggttggcgactcctggataagttttgcaagctgctggtgatcaaagctcatttgcccaaattcatcctgtaaagtctgtaagacttctgacaactcctcattaataccgttggaggagggaggtgttactgacaacttcttacttttaccacctcgtgaagatacttgctttgccaaaggaatactgttgatgactcgatcattgcacaaagctttactgtgttgcttcattagatgcaagacaagctgaacattggctaccacggcatggctagggcttgtggacttcccagctacaaatggcatatcacccaagcataatctataatgtggttgtgcaccaaaatagttcctagaacttttcttttctggtggttttgacttcttttttttaattcttcttgcattgggaacacacggagttgccttatcttcaaagataagtctatttgtttctagaccagtctgcaactcagctgccttagcttgcatgcgtttcctttcctgttcttcttcatggagttttgcttccaactcttgcatttttttttgtttctctaagacagatgtcctctccatttcggcatgctttatcatatttcgcatgtattccaattgtttttctaatagattgcatttattttctgcagctaacaactgagatgtcagttcttgattgtgctttgattcctcattctttgaattctccctttcttgtatctgttcatccagtactttcttatattcaattgtttctctagacaaggttttcacactttcttctgcctgaatcctctcaagttccaagcgtcgaatcttatcttgaagattcttaagagcagaaaatatggctctgctgttgctttctggataggcaagtgtaggcttacttggggagcgtcgtagatcactattaaggaaaggcttatccgaaggatatactacatatggagatgaagaatgccgaaccatgcttccattagaccttgatggctcagcaaagctgttcaatgataagaggtgcacaaatcagaaaataggataccatttcacacacacagcaaaaatttacaagtgggacgataccatccatttaagaggacataaaataaagagggttgttggtataatcacttggtaaaacaatttagtatgaccgagtaaagctgaagacgcacatactctgtgaaccagataattcattcagttatatttgctgaacgattttctctctcttctttcttgaaaatgatacgggttgagtcacagtacatattccatgacccactactgagctgtaatccagagcccagcctctggt

SEQ ID NO: 16845 - RNA, 2133 nt, Homo sapiens
  source 1..2133: mol_type = other RNA
tacgtagatatatatgtatttttaaatatagaaaaactccaccaatagtagaaacaaagtatgtttaatggttgctttggaaaggggaagtgggcacctcatgccagggagatttaaaaatgagacttttcaagcaagcactgcctatagcatagtctcatattttgaaaatttaaacctaattttaattatatataaagaactattttaaaaaatcacacccacaagtaaaaaactggtaatctgtttacaaagtgcagcgtcagtacagcaaactcatctcaacaaaagattatgtgtggtttctcgggctttaaaactcccctggtttccatttaaatgctttaacattgagtcatcctgcatacatgaaaagcctgtgtaatgaagcctgggtcctttaacacctgctattaattaattccaacataagtgagtatgagacctgggaagtaaattgtcatcatctgattgatgaggtacagattatctgaataaaatttctgacctggttatgagtcagtaatcccaacacaaactactgctttgtaatgaattctgtatgctttgcatgtccttcaataactgaagattttttctccttttttctccaggtctcagtttcataaaatctttcttatttgtggtccctgtgattccagaacggctgctgctgtttctttcttcatcaagagtctttttggtagcttttaattccttcttctgcttctctaacttctgtttctccagctgggcttggtattttcgaactttagttatttggttggcttttgcttccatccttcccactaatgcctccaattcacactccaacttgtctttcagttcaacggttggcgactcctggataagttttgcaagctgctggtgatcaaagctcatttgcccaaattcatcctgtaaagtctgtaagacttctgacaactcctcattaataccgttggaggagggaggtgttactgacaacttcttacttttaccacctcgtgaagatacttgctttgccaaaggaatactgttgatgactcgatcattgcacaaagctttactgtgttgcttcattagatgcaagacaagctgaacattggctaccacggcatggctagggcttgtggacttcccagctacaaatggcatatcacccaagcataatctataatgtggttgtgcaccaaaatagttcctagaacttttcttttctggtggttttgacttcttttttttaattcttcttgcattgggaacacacggagttgccttatcttcaaagataagtctatttgtttctagaccagtctgcaactcagctgccttagcttgcatgcgtttcctttcctgttcttcttcatggagttttgcttccaactcttgcatttttttttgtttctctaagacagatgtcctctccatttcggcatgctttatcatatttcgcatgtattccaattgtttttctaatagattgcatttattttctgcagctaacaactgagatgtcagttcttgattgtgctttgattcctcattctttgaattctccctttcttgtatctgttcatccagtactttcttatattcaattgtttctctagacaaggttttcacactttcttctgcctgaatcctctcaagttccaagcgtcgaatcttatcttgaagattcttaagagcagaaaatatggctctgctgttgctttctggataggcaagtgtaggcttacttggggagcgtcgtagatcactattaaggaaaggcttatccgaaggatatactacatatggagatgaagaatgccgaaccatgcttccattagaccttgatggctcagcaaagctgttcgacaagtgagaaccagaagccgcagagacagacgccgccgccatctttcagcctgcccagggggtctccgcacttcgggggcggtctaggttctcgtgctcttctccaagactcgggagccgcccaccagcggggaccctaggctgaacccctgatggaaaagggcaagggtgctggtgctgggcttggaaacccctgcaacacaccccctcagggccgcctacgctcacagcttacacagaaagggcaacacgtcctaacggacgtctttc

SEQ ID NO: 16846 - RNA, 2145 nt, Homo sapiens
  source 1..2145: mol_type = other RNA
tacgtagatatatatgtatttttaaatatagaaaaactccaccaatagtagaaacaaagtatgtttaatggttgctttggaaaggggaagtgggcacctcatgccagggagatttaaaaatgagacttttcaagcaagcactgcctatagcatagtctcatattttgaaaatttaaacctaattttaattatatataaagaactattttaaaaaatcacacccacaagtaaaaaactggtaatctgtttacaaagtgcagcgtcagtacagcaaactcatctcaacaaaagattatgtgtggtttctcgggctttaaaactcccctggtttccatttaaatgctttaacattgagtcatcctgcatacatgaaaagcctgtgtaatgaagcctgggtcctttaacacctgctattaattaattccaacataagtgagtatgagacctgggaagtaaattgtcatcatctgattgatgaggtacagattatctgaataaaatttctgacctggttatgagtcagtaatcccaacacaaactactgctttgtaatgaattctgtatgctttgcatgtccttcaataactgaagattttttctccttttttctccaggtctcagtttcataaaatctttcttatttgtggtccctgtgattccagaacggctgctgctgtttctttcttcatcaagagtctttttggtagcttttaattccttcttctgcttctctaacttctgtttctccagctgggcttggtattttcgaactttagttatttggttggcttttgcttccatccttcccactaatgcctccaattcacactccaacttgtctttcagttcaacggttggcgactcctggataagttttgcaagctgctggtgatcaaagctcatttgcccaaattcatcctgtaaagtctgtaagacttctgacaactcctcattaataccgttggaggagggaggtgttactgacaacttcttacttttaccacctcgtgaagatacttgctttgccaaaggaatactgttgatgactcgatcattgcacaaagctttactgtgttgcttcattagatgcaagacaagctgaacattggctaccacggcatggctagggcttgtggacttttctggtggttttgacttcttttttttaattcttcttgcattgggaacacacggagttgccttatcttcaaagataagtctatttgtttctagaccagtctgcaactcagctgccttagcttgcatgcgtttcctttcctgttcttcttcatggagttttgcttccaactcttgcatttttttttctgcaagggcctgcattgtggtaagtttgttatactcctgttcaagaagatccaatttttcaagttggctctgaacatgtgtttgatcatgttgtcgttctctttctagggaaacttgtttctctaagacagatgtcctctccatttcggcatgctttatcatatttcgcatgtattccaattgtttttctaatagattgcatttattttctgcagctaacaactgagatgtcagttcttgattgtgctttgattcctcattctttgaattctccctttcttgtatctgttcatccagtactttcttatattcaattgtttctctagacaaggttttcacactttcttctgcctgaatcctctcaagttccaagcgtcgaatcttatcttgaagattcttaagagcagaaaatatggctctgctgttgctttctggataggcaagtgtaggcttacttggggagcgtcgtagatcactattaaggaaaggcttatccgaaggatatactacatatggagatgaagaatgccgaaccatgcttccattagaccttgatggctcagcaaagctgttcgacaagtgagaaccagaagccgcagagacagacgccgccgccatctttcagcctgcccagggggtctccgcacttcgggggcggtctaggttctcgtgctcttctccaagactcgggagccgcccaccagcggggaccctaggctgaacccctgatggaaaagggcaagggtgctggtgctgggcttggaaacccctgcaacacaccccctcagggccgcctacgctcacagcttacacagaaag

SEQ ID NO: 16847 - RNA, 2055 nt, Homo sapiens
  source 1..2055: mol_type = other RNA
tacgtagatatatatgtatttttaaatatagaaaaactccaccaatagtagaaacaaagtatgtttaatggttgctttggaaaggggaagtgggcacctcatgccagggagatttaaaaatgagacttttcaagcaagcactgcctatagcatagtctcatattttgaaaatttaaacctaattttaattatatataaagaactattttaaaaaatcacacccacaagtaaaaaactggtaatctgtttacaaagtgcagcgtcagtacagcaaactcatctcaacaaaagattatgtgtggtttctcgggctttaaaactcccctggtttccatttaaatgctttaacattgagtcatcctgcatacatgaaaagcctgtgtaatgaagcctgggtcctttaacacctgctattaattaattccaacataagtgagtatgagacctgggaagtaaattgtcatcatctgattgatgaggtacagattatctgaataaaatttctgacctggttatgagtcagtaatcccaacacaaactactgctttgtaatgaattctgtatgctttgcatgtccttcaataactgaagattttttctccttttttctccaggtctcagtttcataaaatctttcttatttgtggtccctgtgattccagaacggctgctgctgtttctttcttcatcaagagtctttttggtagcttttaattccttcttctgcttctctaacttctgtttctccagctgggcttggtattttcgaactttagttatttggttggcttttgcttccatccttcccactaatgcctccaattcacactccaacttgtctttcagttcaacggttggcgactcctggataagttttgcaagctgctggtgatcaaagctcatttgcccaaattcatcctgtaaagtctgtaagacttctgacaactcctcattaataccgttggaggagggaggtgttactgacaacttcttacttttaccacctcgtgaagatacttgctttgccaaaggaatactgttgatgactcgatcattgcacaaagctttactgtgttgcttcattagatgcaagacaagctgaacattggctaccacggcatggctagggcttgtggacttttctggtggttttgacttcttttttttaattcttcttgcattgggaacacacggagttgccttatcttcaaagataagtctatttgtttctagaccagtctgcaactcagctgccttagcttgcatgcgtttcctttcctgttcttcttcatggagttttgcttccaactcttgcatttttttttgtttctctaagacagatgtcctctccatttcggcatgctttatcatatttcgcatgtattccaattgtttttctaatagattgcatttattttctgcagctaacaactgagatgtcagttcttgattgtgctttgattcctcattctttgaattctccctttcttgtatctgttcatccagtactttcttatattcaattgtttctctagacaaggttttcacactttcttctgcctgaatcctctcaagttccaagcgtcgaatcttatcttgaagattcttaagagcagaaaatatggctctgctgttgctttctggataggcaagtgtaggcttacttggggagcgtcgtagatcactattaaggaaaggcttatccgaaggatatactacatatggagatgaagaatgccgaaccatgcttccattagaccttgatggctcagcaaagctgttcgacaagtgagaaccagaagccgcagagacagacgccgccgccatctttcagcctgcccagggggtctccgcacttcgggggcggtctaggttctcgtgctcttctccaagactcgggagccgcccaccagcggggaccctaggctgaacccctgatggaaaagggcaagggtgctggtgctgggcttggaaacccctgcaacacaccccctcagggccgcctacgctcacagcttacacagaaagggcaacacgtcctaacggacgtctttc

SEQ ID NO: 16848 - RNA, 2967 nt, Homo sapiens
  source 1..2967: mol_type = other RNA
tacgtagatatatatgtatttttaataaagtctctcacttgcttcaaaatttaaggatgatctttttcctggtcagtcatttcaagggaacaataaataaagtagaaaaggatgaactgttttgcatatttctgtggaagaacggaaaacatactttgagaggttcggaaaattcactgtacagaatgaacagcttatatacactatctgtgcaatttttcttggctggggtatttaaatgcaagagctcctccaaaataagaagccacattcattcttgtccaaatccctctgtctcttctattgcaaaaagaagtttttcctttagttgttcataactcttatatggtggtagatccaagcgattaaaacatgtatggcttcttggtaaccaagtgtctttgccaactttttcaatgcaaaacttttgaggcccattacttcccatgagctcagcaaatcctcctagaggtaaacggcaggttccagtgacgaactgcaatagtcgcattcttacttcattgtctgtctctttcacaaactgccaaaaccaaatgatttgcttgctgtttcttgtataatgtcgataaacagtatttctctgccaatctgccaagtcaacctcctgcatgccacacaacataacctctaattctttttcatcgaagtactgtagccactgaagaggaacaacttcattaaaaccatcaaggaaagctttggtctgttcttgtactcctcgagaaaaacgccattctgtcattaaaccaatatattcatctttgttctcctcagtcaccagaatattggaacctcccaacttcaggtcatgtgaagtaacttttcccaaaatctccatgtcaacagaaaagtacatttctaagccacattcttcaatgttgttatctcttatccagataagggagttataaaattcagtatcaatagattccaaatccttaatagtaagttttttacttaacatacgcttgtagaatggtaaagagaaaccagtatcgataaactttccatgaaatagtgccatggcaataaaacgaccaatgaaacagaagtatgaaagatggtctggattaatggttgatgctggatttatctgcagacaatagttgttcttgcccgcatactcaaataagcaatacattgggttcaaaacttcatgtgaaagcaagaaaaaccattctctcgctaggccaccataatcaagtccttcttctcctctaaatattacatataagcgcctcctcaagtcatagggttttaatgccataatctggcacaaataacggaagtgagcaagcttccacctaaagccgcgttcataagcaatttgtggaccacctttagttacagatgacttcccattgcgaggatctttgaatgttgttgttcttgtgttatgatcaacaaagtaccttacaccttcacgagtatatctaatttcccagccttctggcaggggttcttcattctgtaagccttgagttcttggatcttcccactgggttgtttttgtgttatgattcacaaagtaaaccctgtctgttgaatccactcttttttcccagcctggtggcaaaggtccataagggtcattttctgcagctaacattgaagccgaatagaggtatcgttggttaaactgttgcatagctccctgcaattggttccgctgagattgccactgttcaaaatttcggacagattccatggtaggccgctgccacgttgttgttctggtgttatgatccacataataaactcttctacgatcatcaactcttctttcccaacctggaggtaaaggttgtggtctctcccatgtggtagttcgagtattatgatccacataataggttctaccatgaggatcttttctttgttcccaccctgatggcaaggtttctgtgttggcattcccagactgctgccgtacaggatccatacacccatctggctgtcttgatttggctgcttcaaaagcagaactacttctagaattagaggtgtcaggctctaatatacttctagcttcagattccaattctgcactggtagaaggaatacattcattgttttctgaggaagtcagtatttcttgaactggaggatcttcaacagtagtactagtgcaatttggagacaaggcattttcttcagacactactggagtacccgtgacagacgcattatcagttggtgcaaatgaggatgattctccattaacagtgtcatcggcaggctcagatgcgagtggttttggagctggtgtatttttgggtctggcagcaacctgagacggagatgaaggtgtgttgtctccattaactacatacgagcagcatgagttttggactagagtgcttgtaggtacatgattatctattccattcgtgccttcaacagccaacattttctattgtgtatcaacagagcttgtttcaaatctatcgttgcttttcctaataaagcatctgcttttaaagtgcgatggctccaaacttgaaattccaatgtagtctgtggcgtaacatttacagttagctgttcatcccattttggattagaagaactactggattttgctgttttcgtaatttctccatctacaactacttctgtatatattgctgttccgaaccagttcttttttcttttaagtttggcactagaaacagttacctgtaactgcaaccttccactgtggttattactagtatcagaccttggtgaagcagtggccatgtcccaaaattcagctaaaacccggcgcgaagctgtcggctcccggcagccgggcggccacggcagcggcacctcctcctgcggcgggcgccctcacccttccgcgcccaagatcgccatctcgcagcaggcgcggcggcagcagccacccaggcgtcggccccggcagcccaggccgccagcagccactcggaacccgcacgc

SEQ ID NO: 16849 - RNA, 3199 nt, Homo sapiens
  source 1..3199: mol_type = other RNA
tacgtagatatatatgtatttttaataaagtctctcacttgcttcaaaatttaaggatgatctttttcctggtcagtcatttcaagggaacaataaataaagtagaaaaggatgaactgttttgcatatttctgtggaagaacggaaaacatactttgagaggttcggaaaattcactgtacagaatgaacagcttatatacactatctgtgcaatttttcttggctggggtatttaaatgcaagagctcctccaaaataagaagccacattcattcttgtccaaatccctctgtctcttctattgcaaaaagaagtttttcctttagttgttcataactcttatatggtggtagatccaagcgattaaaacatgtatggcttcttggtaaccaagtgtctttgccaactttttcaatgcaaaacttttgaggcccattacttcccatgagctcagcaaatcctcctagaggtaaacggcaggttccagtgacgaactgcaatagtcgcattcttacttcattgtctgtctctttcacaaactgccaaaaccaaatgatttgcttgctgtttcttgtataatgtcgataaacagtatttctctgccaatctgccaagtcaacctcctgcatgccacacaacataacctctaattctttttcatcgaagtactgtagccactgaagaggaacaacttcattaaaaccatcaaggaaagctttggtctgttcttgtactcctcgagaaaaacgccattctgtcattaaaccaatatattcatctttgttctcctcagtcaccagaatattggaacctcccaacttcaggtcatgtgaagtaacttttcccaaaatctccatgtcaacagaaaagtacatttctaagccacattcttcaatgttgttatctcttatccagataagggagttataaaattcagtatcaatagattccaaatccttaatagtaagttttttacttaacatacgcttgtagaatggtaaagagaaaccagtatcgataaactttccatgaaatagtgccatggcaataaaacgaccaatgaaacagaagtatgaaagatggtctggattaatggttgatgctggatttatctgcagacaatagttgttcttgcccgcatactcaaataagcaatacattgggttcaaaacttcatgtgaaagcaagaaaaaccattctctcgctaggccaccataatcaagtccttcttctcctctaaatattacatataagcgcctcctcaagtcatagggttttaatgccataatctggcacaaataacggaagtgagcaagcttccacctaaagccgcgttcataagcaatttgtggaccacctttagttacagatgacttcccattgcgaggatctttgaatgttgttgttcttgtgttatgatcaacaaagtaccttacaccttcacgagtatatctaatttcccagccttctggcaggggttcttcattctgtaagccttgagttcttggatcttcccactgggttgtttttgtgttatgattcacaaagtaaaccctgtctgttgaatccactcttttttcccagcctggtggcaaaggtccataagggtcattttctgcagctaacattgaagccgaatagaggtatcgttggttaaactgttgcatagctccctgcaattggttccgctgagattgccactgttcaaaatttcggacagattccatggtaggccgctgccacgttgttgttctggtgttatgatccacataataaactcttctacgatcatcaactcttctttcccaacctggaggtaaaggttgtggtctctcccatgtggtagttcgagtattatgatccacataataggttctaccatgaggatcttttctttgttcccaccctgatggcaaggtttctgtgttggcattcccagactgctgccgtacaggatccatacacccatctggctgtcttgatttggctgcttcaaaagcagaactacttctagaattagaggtgtcaggctctaatatacttctagcttcagattccaattctgcactggtagaaggaatacattcattgttttctgaggaagtcagtatttcttgaactggaggatcttcaacagtagtactagtgcaatttggagacaaggcattttcttcagacactactggagtacccgtgacagacgcattatcagttggtgcaaatgaggatgattctccattaacagtgtcatcggcaggctcagatgcgagtggttttggagctggtgtatttttgggtctggcagcaacctgagacggagatgaaggtgtgttgtctccattaactacatacgagcagcatgagttttggactagagtgcttgtaggtacatgattatctattccattcgtgccttcaacagccaacctggcagttgtccttgctgaaggctctccattttcatgtaaggcatcaccattttcctgtatttctatggttggagatgagctgcagtttgttatattttcttgctcaatcaccaatccatcaagcacaactgtcaattcaccagtttgtgctatgccattcttgttttccaaggaaagttttaattgttctttcactctttccaattttctattgtgtatcaacagagcttgtttcaaatctatcgttgcttttcctaataaagcatctgcttttaaagtgcgatggctccaaacttgaaattccaatgtagtctgtggcgtaacatttacagttagctgttcatcccattttggattagaagaactactggattttgctgttttcgtaatttctccatctacaactacttctgtatatattgctgttccgaaccagttcttttttcttttaagtttggcactagaaacagttacctgtaactgcaaccttccactgtggttattactagtatcagaccttggtgaagcagtggccatgtcccaaaattcagctaaaacccggcgcgaagctgtcggctcccggcagccgggcggccacggcagcggcacctcctcctgcggcgggcgccctcacccttccgcgcccaagatcgccatctcgcagcaggcgcggcggcagcagccacccaggcgtcggccccggcagcccaggccgccagcagccactcggaacccgcacgcggagctcgccgacacccgaccctcccc

SEQ ID NO: 16850 - RNA, 3235 nt, Homo sapiens
  source 1..3235: mol_type = other RNA
tacgtagatatatatgtatttttaataaagtctctcacttgcttcaaaatttaaggatgatctttttcctggtcagtcatttcaagggaacaataaataaagtagaaaaggatgaactgttttgcatatttctgtggaagaacggaaaacatactttgagaggttcggaaaattcactgtacagaatgaacagcttatatacactatctgtgcaatttttcttggctggggtatttaaatgcaagagctcctccaaaataagaagccacattcattcttgtccaaatccctctgtctcttctattgcaaaaagaagtttttcctttagttgttcataactcttatatggtggtagatccaagcgattaaaacatgtatggcttcttggtaaccaagtgtctttgccaactttttcaatgcaaaacttttgaggcccattacttcccatgagctcagcaaatcctcctagaggtaaacggcaggttccagtgacgaactgcaatagtcgcattcttacttcattgtctgtctctttcacaaactgccaaaaccaaatgatttgcttgctgtttcttgtataatgtcgataaacagtatttctctgccaatctgccaagtcaacctcctgcatgccacacaacataacctctaattctttttcatcgaagtactgtagccactgaagaggaacaacttcattaaaaccatcaaggaaagctttggtctgttcttgtactcctcgagaaaaacgccattctgtcattaaaccaatatattcatctttgttctcctcagtcaccagaatattggaacctcccaacttcaggtcatgtgaagtaacttttcccaaaatctccatgtcaacagaaaagtacatttctaagccacattcttcaatgttgttatctcttatccagataagggagttataaaattcagtatcaatagattccaaatccttaatagtaagttttttacttaacatacgcttgtagaatggtaaagagaaaccagtatcgataaactttccatgaaatagtgccatggcaataaaacgaccaatgaaacagaagtatgaaagatggtctggattaatggttgatgctggatttatctgcagacaatagttgttcttgcccgcatactcaaataagcaatacattgggttcaaaacttcatgtgaaagcaagaaaaaccattctctcgctaggccaccataatcaagtccttcttctcctctaaatattacatataagcgcctcctcaagtcatagggttttaatgccataatctggcacaaataacggaagtgagcaagcttccacctaaagccgcgttcataagcaatttgtggaccacctttagttacagatgacttcccattgcgaggatctttgaatgttgttgttcttgtgttatgatcaacaaagtaccttacaccttcacgagtatatctaatttcccagccttctggcaggggttcttcattctgtaagccttgagttcttggatcttcccactgggttgtttttgtgttatgattcacaaagtaaaccctgtctgttgaatccactcttttttcccagcctggtggcaaaggtccataagggtcattttctgcagctaacattgaagccgaatagaggtatcgttggttaaactgttgcatagctccctgcaattggttccgctgagattgccactgttcaaaatttcggacagattccatggtaggccgctgccacgttgttgttctggtgttatgatccacataataaactcttctacgatcatcaactcttctttcccaacctggaggtaaaggttgtggtctctcccatgtggtagttcgagtattatgatccacataataggttctaccatgaggatcttttctttgttcccaccctgatggcaaggtttctgtgttggcattcccagactgctgccgtacaggatccatacacccatctggctgtcttgatttggctgcttcaaaagcagaactacttctagaattagaggtgtcaggctctaatatacttctagcttcagattccaattctgcactggtagaaggaatacattcattgttttctgaggaagtcagtatttcttgaactggaggatcttcaacagtagtactagtgcaatttggagacaaggcattttcttcagacactactggagtacccgtgacagacgcattatcagttggtgcaaatgaggatgattctccattaacagtgtcatcggcaggctcagatgcgagtggttttggagctggtgtatttttgggtctggcagcaacctgagacggagatgaaggtgtgttgtctccattaactacatacgagcagcatgagttttggactagagtgcttgtaggtacatgattatctattccattcgtgccttcaacagccaacctggcagttgtccttgctgaaggctctccattttcatgtaaggcatcaccattttcctgtatttctatggttggagatgagctgcagtttgttatattttcttgctcaatcaccaatccatcaagcacaactgtcaattcaccagtttgtgctatgccattcttgttttccaaggaaagttttaattgttctttcactctttccaattttctattgtgtatcaacagagcttgtttcaaatctatcgttgcttttcctaataaagcatctgcttttaaagtgcgatggctccaaacttgaaattccaatgtagtctgtggcgtaacatttacagttagctgttcatcccattttggattagaagaactactggattttgctgttttcgtaatttctccatctacaactacttctgtatatattgctgttccgaaccagttcttttttcttttaagtttggcactagaaacagttacctgtaactgcaaccttccactgtggttattactagtatcagaccttggtgaagcagtggccatgtcccaaaattcagctaaaactatgtatcaggaactgctagacactggggatacaaagatgagtaagacacgattccctctttcaaggagctcatagtctgtgaggagacaaccccggcgcgaagctgtcggctcccggcagccgggcggccacggcagcggcacctcctcctgcggcgggcgccctcacccttccgcgcccaagatcgccatctcgcagcaggcgcggcggcagcagccacccaggcgtcggccccggcagcccag

SEQ ID NO: 16851 - RNA, 3318 nt, Homo sapiens
  source 1..3318: mol_type = other RNA
tacgtagatatatatgtatttttaataaagtctctcacttgcttcaaaatttaaggatgatctttttcctggtcagtcatttcaagggaacaataaataaagtagaaaaggatgaactgttttgcatatttctgtggaagaacggaaaacatactttgagaggttcggaaaattcactgtacagaatgaacagcttatatacactatctgtgcaatttttcttggctggggtatttaaatgcaagagctcctccaaaataagaagccacattcattcttgtccaaatccctctgtctcttctattgcaaaaagaagtttttcctttagttgttcataactcttatatggtggtagatccaagcgattaaaacatgtatggcttcttggtaaccaagtgtctttgccaactttttcaatgcaaaacttttgaggcccattacttcccatgagctcagcaaatcctcctagaggtaaacggcaggttccagtgacgaactgcaatagtcgcattcttacttcattgtctgtctctttcacaaactgccaaaaccaaatgatttgcttgctgtttcttgtataatgtcgataaacagtatttctctgccaatctgccaagtcaacctcctgcatgccacacaacataacctctaattctttttcatcgaagtactgtagccactgaagaggaacaacttcattaaaaccatcaaggaaagctttggtctgttcttgtactcctcgagaaaaacgccattctgtcattaaaccaatatattcatctttgttctcctcagtcaccagaatattggaacctcccaacttcaggtcatgtgaagtaacttttcccaaaatctccatgtcaacagaaaagtacatttctaagccacattcttcaatgttgttatctcttatccagataagggagttataaaattcagtatcaatagattccaaatccttaatagtaagttttttacttaacatacgcttgtagaatggtaaagagaaaccagtatcgataaactttccatgaaatagtgccatggcaataaaacgaccaatgaaacagaagtatgaaagatggtctggattaatggttgatgctggatttatctgcagacaatagttgttcttgcccgcatactcaaataagcaatacattgggttcaaaacttcatgtgaaagcaagaaaaaccattctctcgctaggccaccataatcaagtccttcttctcctctaaatattacatataagcgcctcctcaagtcatagggttttaatgccataatctgttggaaggaatcttcaaacaatgtctgccgggacacattgatctttacatgactaggtagtgcattagacactatagtacctggcacaaataacggaagtgagcaagcttccacctaaagccgcgttcataagcaatttgtggaccacctttagttacagatgacttcccattgcgaggatctttgaatgttgttgttcttgtgttatgatcaacaaagtaccttacaccttcacgagtatatctaatttcccagccttctggcaggggttcttcattctgtaagccttgagttcttggatcttcccactgggttgtttttgtgttatgattcacaaagtaaaccctgtctgttgaatccactcttttttcccagcctggtggcaaaggtccataagggtcattttctgcagctaacattgaagccgaatagaggtatcgttggttaaactgttgcatagctccctgcaattggttccgctgagattgccactgttcaaaatttcggacagattccatggtaggccgctgccacgttgttgttctggtgttatgatccacataataaactcttctacgatcatcaactcttctttcccaacctggaggtaaaggttgtggtctctcccatgtggtagttcgagtattatgatccacataataggttctaccatgaggatcttttctttgttcccaccctgatggcaaggtttctgtgttggcattcccagactgctgccgtacaggatccatacacccatctggctgtcttgatttggctgcttcaaaagcagaactacttctagaattagaggtgtcaggctctaatatacttctagcttcagattccaattctgcactggtagaaggaatacattcattgttttctgaggaagtcagtatttcttgaactggaggatcttcaacagtagtactagtgcaatttggagacaaggcattttcttcagacactactggagtacccgtgacagacgcattatcagttggtgcaaatgaggatgattctccattaacagtgtcatcggcaggctcagatgcgagtggttttggagctggtgtatttttgggtctggcagcaacctgagacggagatgaaggtgtgttgtctccattaactacatacgagcagcatgagttttggactagagtgcttgtaggtacatgattatctattccattcgtgccttcaacagccaacctggcagttgtccttgctgaaggctctccattttcatgtaaggcatcaccattttcctgtatttctatggttggagatgagctgcagtttgttatattttcttgctcaatcaccaatccatcaagcacaactgtcaattcaccagtttgtgctatgccattcttgttttccaaggaaagttttaattgttctttcactctttccaattttctattgtgtatcaacagagcttgtttcaaatctatcgttgcttttcctaataaagcatctgcttttaaagtgcgatggctccaaacttgaaattccaatgtagtctgtggcgtaacatttacagttagctgttcatcccattttggattagaagaactactggattttgctgttttcgtaatttctccatctacaactacttctgtatatattgctgttccgaaccagttcttttttcttttaagtttggcactagaaacagttacctgtaactgcaaccttccactgtggttattactagtatcagaccttggtgaagcagtggccatgtcccaaaattcagctaaaactatgtatcaggaactgctagacactggggatacaaagatgagtaagacacgattccctctttcaaggagctcatagtctgtgaggagacaaccccggcgcgaagctgtcggctcccggcagccgggcggccacggcagcggcacctcctcctgcggcgggcgccctcacccttccgcgcccaagatcgccatctcgcagcaggcgcggcggcagcagccacccaggcgtcggccccggcagcccag

SEQ ID NO: 16852 - RNA, 3060 nt, Homo sapiens
  source 1..3060: mol_type = other RNA
tacgtagatatatatgtatttttaataaagtctctcacttgcttcaaaatttaaggatgatctttttcctggtcagtcatttcaagggaacaataaataaagtagaaaaggatgaactgttttgcatatttctgtggaagaacggaaaacatactttgagaggttcggaaaattcactgtacagaatgaacagcttatatacactatctgtgcaatttttcttggctggggtatttaaatgcaagagctcctccaaaataagaagccacattcattcttgtccaaatccctctgtctcttctattgcaaaaagaagtttttcctttagttgttcataactcttatatggtggtagatccaagcgattaaaacatgtatggcttcttggtaaccaagtgtctttgccaactttttcaatgcaaaacttttgaggcccattacttcccatgagctcagcaaatcctcctagaggtaaacggcaggttccagtgacgaactgcaatagtcgcattcttacttcattgtctgtctctttcacaaactgccaaaaccaaatgatttgcttgctgtttcttgtataatgtcgataaacagtatttctctgccaatctgccaagtcaacctcctgcatgccacacaacataacctctaattctttttcatcgaagtactgtagccactgaagaggaacaacttcattaaaaccatcaaggaaagctttggtctgttcttgtactcctcgagaaaaacgccattctgtcattaaaccaatatattcatctttgttctcctcagtcaccagaatattggaacctcccaacttcaggtcatgtgaagtaacttttcccaaaatctccatgtcaacagaaaagtacatttctaagccacattcttcaatgttgttatctcttatccagataagggagttataaaattcagtatcaatagattccaaatccttaatagtaagttttttacttaacatacgcttgtagaatggtaaagagaaaccagtatcgataaactttccatgaaatagtgccatggcaataaaacgaccaatgaaacagaagtatgaaagatggtctggattaatggttgatgctggatttatctgcagacaatagttgttcttgcccgcatactcaaataagcaatacattgggttcaaaacttcatgtgaaagcaagaaaaaccattctctcgctaggccaccataatcaagtccttcttctcctctaaatattacatataagcgcctcctcaagtcatagggttttaatgccataatctgttggaaggaatcttcaaacaatgtctgccgggacacattgatctttacatgactaggtagtgcattagactggcacaaataacggaagtgagcaagcttccacctaaagccgcgttcataagcaatttgtggaccacctttagttacagatgacttcccattgcgaggatctttgaatgttgttgttcttgtgttatgatcaacaaagtaccttacaccttcacgagtatatctaatttcccagccttctggcaggggttcttcattctgtaagccttgagttcttggatcttcccactgggttgtttttgtgttatgattcacaaagtaaaccctgtctgttgaatccactcttttttcccagcctggtggcaaaggtccataagggtcattttctgcagctaacattgaagccgaatagaggtatcgttggttaaactgttgcatagctccctgcaattggttccgctgagattgccactgttcaaaatttcggacagattccatggtaggccgctgccacgttgttgttctggtgttatgatccacataataaactcttctacgatcatcaactcttctttcccaacctggaggtaaaggttgtggtctctcccatgtggtagttcgagtattatgatccacataataggttctaccatgaggatcttttctttgttcccaccctgatggcaaggtttctgtgttggcattcccagactgctgccgtacaggatccatacacccatctggctgtcttgatttggctgcttcaaaagcagaactacttctagaattagaggtgtcaggctctaatatacttctagcttcagattccaattctgcactggtagaaggaatacattcattgttttctgaggaagtcagtatttcttgaactggaggatcttcaacagtagtactagtgcaatttggagacaaggcattttcttcagacactactggagtacccgtgacagacgcattatcagttggtgcaaatgaggatgattctccattaacagtgtcatcggcaggctcagatgcgagtggttttggagctggtgtatttttgggtctggcagcaacctgagacggagatgaaggtgtgttgtctccattaactacatacgagcagcatgagttttggactagagtgcttgtaggtacatgattatctattccattcgtgccttcaacagccaacattttctattgtgtatcaacagagcttgtttcaaatctatcgttgcttttcctaataaagcatctgcttttaaagtgcgatggctccaaacttgaaattccaatgtagtctgtggcgtaacatttacagttagctgttcatcccattttggattagaagaactactggattttgctgttttcgtaatttctccatctacaactacttctgtatatattgctgttccgaaccagttcttttttcttttaagtttggcactagaaacagttacctgtaactgcaaccttccactgtggttattactagtatcagaccttggtgaagcagtggccatgtcccaaaattcagctaaaacccggcgcgaagctgtcggctcccggcagccgggcggccacggcagcggcacctcctcctgcggcgggcgccctcacccttccgcgcccaagatcgccatctcgcagcaggcgcggcggcagcagccacccaggcgtcggccccggcagcccaggccgccagcagccactcggaacccgcacgcggagctcgccgacacccgacc

SEQ ID NO: 16853 - RNA, 3102 nt, Homo sapiens
  source 1..3102: mol_type = other RNA
tacgtagatatatatgtatttttaataaagtctctcacttgcttcaaaatttaaggatgatctttttcctggtcagtcatttcaagggaacaataaataaagtagaaaaggatgaactgttttgcatatttctgtggaagaacggaaaacatactttgagaggttcggaaaattcactgtacagaatgaacagcttatatacactatctgtgcaatttttcttggctggggtatttaaatgcaagagctcctccaaaataagaagccacattcattcttgtccaaatccctctgtctcttctattgcaaaaagaagtttttcctttagttgttcataactcttatatggtggtagatccaagcgattaaaacatgtatggcttcttggtaaccaagtgtctttgccaactttttcaatgcaaaacttttgaggcccattacttcccatgagctcagcaaatcctcctagaggtaaacggcaggttccagtgacgaactgcaatagtcgcattcttacttcattgtctgtctctttcacaaactgccaaaaccaaatgatttgcttgctgtttcttgtataatgtcgataaacagtatttctctgccaatctgccaagtcaacctcctgcatgccacacaacataacctctaattctttttcatcgaagtactgtagccactgaagaggaacaacttcattaaaaccatcaaggaaagctttggtctgttcttgtactcctcgagaaaaacgccattctgtcattaaaccaatatattcatctttgttctcctcagtcaccagaatattggaacctcccaacttcaggtcatgtgaagtaacttttcccaaaatctccatgtcaacagaaaagtacatttctaagccacattcttcaatgttgttatctcttatccagataagggagttataaaattcagtatcaatagattccaaatccttaatagtaagttttttacttaacatacgcttgtagaatggtaaagagaaaccagtatcgataaactttccatgaaatagtgccatggcaataaaacgaccaatgaaacagaagtatgaaagatggtctggattaatggttgatgctggatttatctgcagacaatagttgttcttgcccgcatactcaaataagcaatacattgggttcaaaacttcatgtgaaagcaagaaaaaccattctctcgctaggccaccataatcaagtccttcttctcctctaaatattacatataagcgcctcctcaagtcatagggttttaatgccataatctgttggaaggaatcttcaaacaatgtctgccgggacacattgatctttacatgactaggtagtgcattagactggcacaaataacggaagtgagcaagcttccacctaaagccgcgttcataagcaatttgtggaccacctttagttacagatgacttcccattgcgaggatctttgaatgttgttgttcttgtgttatgatcaacaaagtaccttacaccttcacgagtatatctaatttcccagccttctggcaggggttcttcattctgtaagccttgagttcttggatcttcccactgggttgtttttgtgttatgattcacaaagtaaaccctgtctgttgaatccactcttttttcccagcctggtggcaaaggtccataagggtcattttctgcagctaacattgaagccgaatagaggtatcgttggttaaactgttgcatagctccctgcaattggttccgctgagattgccactgttcaaaatttcggacagattccatggtaggccgctgccacgttgttgttctggtgttatgatccacataataaactcttctacgatcatcaactcttctttcccaacctggaggtaaaggttgtggtctctcccatgtggtagttcgagtattatgatccacataataggttctaccatgaggatcttttctttgttcccaccctgatggcaaggtttctgtgttggcattcccagactgctgccgtacaggatccatacacccatctggctgtcttgatttggctgcttcaaaagcagaactacttctagaattagaggtgtcaggctctaatatacttctagcttcagattccaattctgcactggtagaaggaatacattcattgttttctgaggaagtcagtatttcttgaactggaggatcttcaacagtagtactagtgcaatttggagacaaggcattttcttcagacactactggagtacccgtgacagacgcattatcagttggtgcaaatgaggatgattctccattaacagtgtcatcggcaggctcagatgcgagtggttttggagctggtgtatttttgggtctggcagcaacctgagacggagatgaaggtgtgttgtctccattaactacatacgagcagcatgagttttggactagagtgcttgtaggtacatgattatctattccattcgtgccttcaacagccaacattttctattgtgtatcaacagagcttgtttcaaatctatcgttgcttttcctaataaagcatctgcttttaaagtgcgatggctccaaacttgaaattccaatgtagtctgtggcgtaacatttacagttagctgttcatcccattttggattagaagaactactggattttgctgttttcgtaatttctccatctacaactacttctgtatatattgctgttccgaaccagttcttttttcttttaagtttggcactagaaacagttacctgtaactgcaaccttccactgtggttattactagtatcagaccttggtgaagcagtggccatgtcccaaaattcagctaaaactatgtatcaggaactgctagacactggggatacaaagatgagtaagacacgattccctctttcaaggagctcatagtctgtgaggagacaaccccggcgcgaagctgtcggctcccggcagccgggcggccacggcagcggcacctcctcctgcggcgggcgccctcacccttccgcgcccaagatcgccatctcgcagcaggcgcggcggcagcagccacccaggcgtcggccccggcagcccag

SEQ ID NO: 16854 - RNA, 3332 nt, Homo sapiens
  source 1..3332: mol_type = other RNA
tacgtagatatatatgtatttttaataaagtctctcacttgcttcaaaatttaaggatgatctttttcctggtcagtcatttcaagggaacaataaataaagtagaaaaggatgaactgttttgcatatttctgtggaagaacggaaaacatactttgagaggttcggaaaattcactgtacagaatgaacagcttatatacactatctgtgcaatttttcttggctggggtatttaaatgcaagagctcctccaaaataagaagccacattcattcttgtccaaatccctctgtctcttctattgcaaaaagaagtttttcctttagttgttcataactcttatatggtggtagatccaagcgattaaaacatgtatggcttcttggtaaccaagtgtctttgccaactttttcaatgcaaaacttttgaggcccattacttcccatgagctcagcaaatcctcctagaggtaaacggcaggttccagtgacgaactgcaatagtcgcattcttacttcattgtctgtctctttcacaaactgccaaaaccaaatgatttgcttgctgtttcttgtataatgtcgataaacagtatttctctgccaatctgccaagtcaacctcctgcatgccacacaacataacctctaattctttttcatcgaagtactgtagccactgaagaggaacaacttcattaaaaccatcaaggaaagctttggtctgttcttgtactcctcgagaaaaacgccattctgtcattaaaccaatatattcatctttgttctcctcagtcaccagaatattggaacctcccaacttcaggtcatgtgaagtaacttttcccaaaatctccatgtcaacagaaaagtacatttctaagccacattcttcaatgttgttatctcttatccagataagggagttataaaattcagtatcaatagattccaaatccttaatagtaagttttttacttaacatacgcttgtagaatggtaaagagaaaccagtatcgataaactttccatgaaatagtgccatggcaataaaacgaccaatgaaacagaagtatgaaagatggtctggattaatggttgatgctggatttatctgcagacaatagttgttcttgcccgcatactcaaataagcaatacattgggttcaaaacttcatgtgaaagcaagaaaaaccattctctcgctaggccaccataatcaagtccttcttctcctctaaatattacatataagcgcctcctcaagtcatagggttttaatgccataatctgttggaaggaatcttcaaacaatgtctgccgggacacattgatctttacatgactaggtagtgcattagactggcacaaataacggaagtgagcaagcttccacctaaagccgcgttcataagcaatttgtggaccacctttagttacagatgacttcccattgcgaggatctttgaatgttgttgttcttgtgttatgatcaacaaagtaccttacaccttcacgagtatatctaatttcccagccttctggcaggggttcttcattctgtaagccttgagttcttggatcttcccactgggttgtttttgtgttatgattcacaaagtaaaccctgtctgttgaatccactcttttttcccagcctggtggcaaaggtccataagggtcattttctgcagctaacattgaagccgaatagaggtatcgttggttaaactgttgcatagctccctgcaattggttccgctgagattgccactgttcaaaatttcggacagattccatggtaggccgctgccacgttgttgttctggtgttatgatccacataataaactcttctacgatcatcaactcttctttcccaacctggaggtaaaggttgtggtctctcccatgtggtagttcgagtattatgatccacataataggttctaccatgaggatcttttctttgttcccaccctgatggcaaggtttctgtgttggcattcccagactgctgccgtacaggatccatacacccatctggctgtcttgatttggctgcttcaaaagcagaactacttctagaattagaggtgtcaggctctaatatacttctagcttcagattccaattctgcactggtagaaggaatacattcattgttttctgaggaagtcagtatttcttgaactggaggatcttcaacagtagtactagtgcaatttggagacaaggcattttcttcagacactactggagtacccgtgacagacgcattatcagttggtgcaaatgaggatgattctccattaacagtgtcatcggcaggctcagatgcgagtggttttggagctggtgtatttttgggtctggcagcaacctgagacggagatgaaggtgtgttgtctccattaactacatacgagcagcatgagttttggactagagtgcttgtaggtacatgattatctattccattcgtgccttcaacagccaacctggcagttgtccttgctgaaggctctccattttcatgtaaggcatcaccattttcctgtatttctatggttggagatgagctgcagtttgttatattttcttgctcaatcaccaatccatcaagcacaactgtcaattcaccagtttgtgctatgccattcttgttttccaaggaaagttttaattgttctttcactctttccaattttctattgtgtatcaacagagcttgtttcaaatctatcgttgcttttcctaataaagcatctgcttttaaagtgcgatggctccaaacttgaaattccaatgtagtctgtggcgtaacatttacagttagctgttcatcccattttggattagaagaactactggattttgctgttttcgtaatttctccatctacaactacttctgtatatattgctgttccgaaccagttcttttttcttttaagtttggcactagaaacagttacctgtaactgcaaccttccactgtggttattactagtatcagaccttggtgaagcagtggccatgtcccaaaattcagctaaaacccggcgcgaagctgtcggctcccggcagccgggcggccacggcagcggcacctcctcctgcggcgggcgccctcacccttccgcgcccaagatcgccatctcgcagcaggcgcggcggcagcagccacccaggcgtcggccccggcagcccaggccgccagcagccactcggaacccgcacgcggagctcgccgacacccgaccctccccccacccccaccccgtccacgcgccacccccagccgaccccacacctcccttcctcgggagc

SEQ ID NO: 16855 - RNA, 3538 nt, Homo sapiens
  source 1..3538: mol_type = other RNA
tacgtagatatatatgtatttttaataaagtctctcacttgcttcaaaatttaaggatgatctttttcctggtcagtcatttcaagggaacaataaataaagtagaaaaggatgaactgttttgcatatttctgtggaagaacggaaaacatactttgagaggttcggaaaattcactgtacagaatgaacagcttatatacactatctgtgcaatttttcttggctggggtatttaaatgcaagagctcctccaaaataagaagccacattcattcttgtccaaatccctctgtctcttctattgcaaaaagaagtttttcctttagttgttcataactcttatatggtggtagatccaagcgattaaaacatgtatggcttcttggtaaccaagtgtctttgccaactttttcaatgcaaaacttttgaggcccattacttcccatgagctcagcaaatcctcctagaggtaaacggcaggttccagtgacgaactgcaatagtcgcattcttacttcattgtctgtctctttcacaaactgccaaaaccaaatgatttgcttgctgtttcttgtataatgtcgataaacagtatttctctgccaatctgccaagtcaacctcctgcatgccacacaacataacctctaattctttttcatcgaagtactgtagccactgaagaggaacaacttcattaaaaccatcaaggaaagctttggtctgttcttgtactcctcgagaaaaacgccattctgtcattaaaccaatatattcatctttgttctcctcagtcaccagaatattggaacctcccaacttcaggtcatgtgaagtaacttttcccaaaatctccatgtcaacagaaaagtacatttctaagccacattcttcaatgttgttatctcttatccagataagggagttataaaattcagtatcaatagattccaaatccttaatagtaagttttttacttaacatacgcttgtagaatggtaaagagaaaccagtatcgataaactttccatgaaatagtgccatggcaataaaacgaccaatgaaacagaagtatgaaagatggtctggattaatggttgatgctggatttatctgcagacaatagttgttcttgcccgcatactcaaataagcaatacattgggttcaaaacttcatgtgaaagcaagaaaaaccattctctcgctaggccaccataatcaagtccttcttctcctctaaatattacatataagcgcctcctcaagtcatagggttttaatgccataatctgttggaaggaatcttcaaacaatgtctgccgggacacattgatctttacatgactaggtagtgcattagactggcacaaataacggaagtgagcaagcttccacctaaagccgcgttcataagcaatttgtggaccacctttagttacagatgacttcccattgcgaggatctttgaatgttgttgttcttgtgttatgatcaacaaagtaccttacaccttcacgagtatatctaatttcccagccttctggcaggggttcttcattctgtaagccttgagttcttggatcttcccactgggttgtttttgtgttatgattcacaaagtaaaccctgtctgttgaatccactcttttttcccagcctggtggcaaaggtccataagggtcattttctgcagctaacattgaagccgaatagaggtatcgttggttaaactgttgcatagctccctgcaattggttccgctgagattgccactgttcaaaatttcggacagattccatggtaggccgctgccacgttgttgttctggtgttatgatccacataataaactcttctacgatcatcaactcttctttcccaacctggaggtaaaggttgtggtctctcccatgtggtagttcgagtattatgatccacataataggttctaccatgaggatcttttctttgttcccaccctgatggcaaggtttctgtgttggcattcccagactgctgccgtacaggatccatacacccatctggctgtcttgatttggctgcttcaaaagcagaactacttctagaattagaggtgtcaggctctaatatacttctagcttcagattccaattctgcactggtagaaggaatacattcattgttttctgaggaagtcagtatttcttgaactggaggatcttcaacagtagtactagtgcaatttggagacaaggcattttcttcagacactactggagtacccgtgacagacgcattatcagttggtgcaaatgaggatgattctccattaacagtgtcatcggcaggctcagatgcgagtggttttggagctggtgtatttttgggtctggcagcaacctgagacggagatgaaggtgtgttgtctccattaactacatacgagcagcatgagttttggactagagtgcttgtaggtacatgattatctattccattcgtgccttcaacagccaacctggcagttgtccttgctgaaggctctccattttcatgtaaggcatcaccattttcctgtatttctatggttggagatgagctgcagtttgttatattttcttgctcaatcaccaatccatcaagcacaactgtcaattcaccagtttgtgctatgccattcttgttttccaaggaaagttttaattgttctttcactctttccaattttctattgtgtatcaacagagcttgtttcaaatctatcgttgcttttcctaataaagcatctgcttttaaagtgcgatggctccaaacttgaaattccaatgtagtctgtggcgtaacatttacagttagctgttcatcccattttggattagaagaactactggattttgctgttttcgtaatttctccatctacaactacttctgtatatattgctgttccgaaccagttcttttttcttttaagtttggcactagaaacagttacctgtaactgcaaccttccactgtggttattactagtatcagaccttggtgaagcagtggccatgtcccaaaattcagctaaaactatgtatcaggaactgctagacactggggatacaaagatgagtaagacacgattccctctttcaaggagctcatagtctgtgaggagacaaccccggcgcgaagctgtcggctcccggcagccgggcggccacggcagcggcacctcctcctgcggcgggcgccctcacccttccgcgcccaagatcgccatctcgcagcaggcgcggcggcagcagccacccaggcgtcggccccggcagcccaggccgccagcagccactcggaacccgcacgcggagctcgccgacacccgaccctccccccacccccaccccgtccacgcgccacccccagccgaccccacacctcccttcctcgggagcgcgccgcgtggccgcgtcgccggcgccgcgccctaagcgcgcgcctccccgccggccccggcaccgcgcgctacgccgcggccgcccaaagcctccaactccggacccggaat

SEQ ID NO: 16856 - RNA, 3273 nt, Homo sapiens
  source 1..3273: mol_type = other RNA
tacgtagatatatatgtatttttaataaagtctctcacttgcttcaaaatttaaggatgatctttttcctggtcagtcatttcaagggaacaataaataaagtagaaaaggatgaactgttttgcatatttctgtggaagaacggaaaacatactttgagaggttcggaaaattcactgtacagaatgaacagcttatatacactatctgtgcaatttttcttggctggggtatttaaatgcaagagctcctccaaaataagaagccacattcattcttgtccaaatccctctgtctcttctattgcaaaaagaagtttttcctttagttgttcataactcttatatggtggtagatccaagcgattaaaacatgtatggcttcttggtaaccaagtgtctttgccaactttttcaatgcaaaacttttgaggcccattacttcccatgagctcagcaaatcctcctagaggtaaacggcaggttccagtgacgaactgcaatagtcgcattcttacttcattgtctgtctctttcacaaactgccaaaaccaaatgatttgcttgctgtttcttgtataatgtcgataaacagtatttctctgccaatctgccaagtcaacctcctgcatgccacacaacataacctctaattctttttcatcgaagtactgtagccactgaagaggaacaacttcattaaaaccatcaaggaaagctttggtctgttcttgtactcctcgagaaaaacgccattctgtcattaaaccaatatattcatctttgttctcctcagtcaccagaatattggaacctcccaacttcaggtcatgtgaagtaacttttcccaaaatctccatgtcaacagaaaagtacatttctaagccacattcttcaatgttgttatctcttatccagataagggagttataaaattcagtatcaatagattccaaatccttaatagtaagttttttacttaacatacgcttgtagaatggtaaagagaaaccagtatcgataaactttccatgaaatagtgccatggcaataaaacgaccaatgaaacagaagtatgaaagatggtctggattaatggttgatgctggatttatctgcagacaatagttgttcttgcccgcatactcaaataagcaatacattgggttcaaaacttcatgtgaaagcaagaaaaaccattctctcgctaggccaccataatcaagtccttcttctcctctaaatattacatataagcgcctcctcaagtcatagggttttaatgccataatctgttggaaggaatcttcaaacaatgtctgccgggacacattgatctttacatgactaggtagtgcattagactggcacaaataacggaagtgagcaagcttccacctaaagccgcgttcataagcaatttgtggaccacctttagttacagatgacttcccattgcgaggatctttgaatgttgttgttcttgtgttatgatcaacaaagtaccttacaccttcacgagtatatctaatttcccagccttctggcaggggttcttcattctgtaagccttgagttcttggatcttcccactgggttgtttttgtgttatgattcacaaagtaaaccctgtctgttgaatccactcttttttcccagcctggtggcaaaggtccataagggtcattttctgcagctaacattgaagccgaatagaggtatcgttggttaaactgttgcatagctccctgcaattggttccgctgagattgccactgttcaaaatttcggacagattccatggtaggccgctgccacgttgttgttctggtgttatgatccacataataaactcttctacgatcatcaactcttctttcccaacctggaggtaaaggttgtggtctctcccatgtggtagttcgagtattatgatccacataataggttctaccatgaggatcttttctttgttcccaccctgatggcaaggtttctgtgttggcattcccagactgctgccgtacaggatccatacacccatctggctgtcttgatttggctgcttcaaaagcagaactacttctagaattagaggtgtcaggctctaatatacttctagcttcagattccaattctgcactggtagaaggaatacattcattgttttctgaggaagtcagtatttcttgaactggaggatcttcaacagtagtactagtgcaatttggagacaaggcattttcttcagacactactggagtacccgtgacagacgcattatcagttggtgcaaatgaggatgattctccattaacagtgtcatcggcaggctcagatgcgagtggttttggagctggtgtatttttgggtctggcagcaacctgagacggagatgaaggtgtgttgtctccattaactacatacgagcagcatgagttttggactagagtgcttgtaggtacatgattatctattccattcgtgccttcaacagccaacctggcagttgtccttgctgaaggctctccattttcatgtaaggcatcaccattttcctgtattttggttggagatgagctgcagtttgttatattttcttgctcaatcaccaatccatcaagcacaactgtcaattcaccagtttgtgctatgccattcttgttttccaaggaaagttttaattgttctttcactctttccaattttctattgtgtatcaacagagcttgtttcaaatctatcgttgcttttcctaataaagcatctgcttttaaagtgcgatggctccaaacttgaaattccaatgtagtctgtggcgtaacatttacagttagctgttcatcccattttggattagaagaactactggattttgctgttttcgtaatttctccatctacaactacttctgtatatattgctgttccgaaccagttcttttttcttttaagtttggcactagaaacagttacctgtaactgcaaccttccactgtggttattactagtatcagaccttggtgaagcagtggccatgtcccaaaattcagctaaaacccggcgcgaagctgtcggctcccggcagccgggcggccacggcagcggcacctcctcctgcggcgggcgccctcacccttccgcgcccaagatcgccatctcgcagcaggcgcggcggcagcagccacccaggcgtcggccccggcagcccaggccgccagcagccactcggaacccgcacgcggagctcgccgacacccgaccctccccccacc

SEQ ID NO: 16857 - RNA, 3304 nt, Homo sapiens
  source 1..3304: mol_type = other RNA
tacgtagatatatatgtatttttaataaagtctctcacttgcttcaaaatttaaggatgatctttttcctggtcagtcatttcaagggaacaataaataaagtagaaaaggatgaactgttttgcatatttctgtggaagaacggaaaacatactttgagaggttcggaaaattcactgtacagaatgaacagcttatatacactatctgtgcaatttttcttggctggggtatttaaatgcaagagctcctccaaaataagaagccacattcattcttgtccaaatccctctgtctcttctattgcaaaaagaagtttttcctttagttgttcataactcttatatggtggtagatccaagcgattaaaacatgtatggcttcttggtaaccaagtgtctttgccaactttttcaatgcaaaacttttgaggcccattacttcccatgagctcagcaaatcctcctagaggtaaacggcaggttccagtgacgaactgcaatagtcgcattcttacttcattgtctgtctctttcacaaactgccaaaaccaaatgatttgcttgctgtttcttgtataatgtcgataaacagtatttctctgccaatctgccaagtcaacctcctgcatgccacacaacataacctctaattctttttcatcgaagtactgtagccactgaagaggaacaacttcattaaaaccatcaaggaaagctttggtctgttcttgtactcctcgagaaaaacgccattctgtcattaaaccaatatattcatctttgttctcctcagtcaccagaatattggaacctcccaacttcaggtcatgtgaagtaacttttcccaaaatctccatgtcaacagaaaagtacatttctaagccacattcttcaatgttgttatctcttatccagataagggagttataaaattcagtatcaatagattccaaatccttaatagtaagttttttacttaacatacgcttgtagaatggtaaagagaaaccagtatcgataaactttccatgaaatagtgccatggcaataaaacgaccaatgaaacagaagtatgaaagatggtctggattaatggttgatgctggatttatctgcagacaatagttgttcttgcccgcatactcaaataagcaatacattgggttcaaaacttcatgtgaaagcaagaaaaaccattctctcgctaggccaccataatcaagtccttcttctcctctaaatattacatataagcgcctcctcaagtcatagggttttaatgccataatctgttggaaggaatcttcaaacaatgtctgccgggacacattgatctttacatgactaggtagtgcattagactggcacaaataacggaagtgagcaagcttccacctaaagccgcgttcataagcaatttgtggaccacctttagttacagatgacttcccattgcgaggatctttgaatgttgttgttcttgtgttatgatcaacaaagtaccttacaccttcacgagtatatctaatttcccagccttctggcaggggttcttcattctgtaagccttgagttcttggatcttcccactgggttgtttttgtgttatgattcacaaagtaaaccctgtctgttgaatccactcttttttcccagcctggtggcaaaggtccataagggtcattttctgcagctaacattgaagccgaatagaggtatcgttggttaaactgttgcatagctccctgcaattggttccgctgagattgccactgttcaaaatttcggacagattccatggtaggccgctgccacgttgttgttctggtgttatgatccacataataaactcttctacgatcatcaactcttctttcccaacctggaggtaaaggttgtggtctctcccatgtggtagttcgagtattatgatccacataataggttctaccatgaggatcttttctttgttcccaccctgatggcaaggtttctgtgttggcattcccagactgctgccgtacaggatccatacacccatctggctgtcttgatttggctgcttcaaaagcagaactacttctagaattagaggtgtcaggctctaatatacttctagcttcagattccaattctgcactggtagaaggaatacattcattgttttctgaggaagtcagtatttcttgaactggaggatcttcaacagtagtactagtgcaatttggagacaaggcattttcttcagacactactggagtacccgtgacagacgcattatcagttggtgcaaatgaggatgattctccattaacagtgtcatcggcaggctcagatgcgagtggttttggagctggtgtatttttgggtctggcagcaacctgagacggagatgaaggtgtgttgtctccattaactacatacgagcagcatgagttttggactagagtgcttgtaggtacatgattatctattccattcgtgccttcaacagccaacctggcagttgtccttgctgaaggctctccattttcatgtaaggcatcaccattttcctgtattttggttggagatgagctgcagtttgttatattttcttgctcaatcaccaatccatcaagcacaactgtcaattcaccagtttgtgctatgccattcttgttttccaaggaaagttttaattgttctttcactctttccaattttctattgtgtatcaacagagcttgtttcaaatctatcgttgcttttcctaataaagcatctgcttttaaagtgcgatggctccaaacttgaaattccaatgtagtctgtggcgtaacatttacagttagctgttcatcccattttggattagaagaactactggattttgctgttttcgtaatttctccatctacaactacttctgtatatattgctgttccgaaccagttcttttttcttttaagtttggcactagaaacagttacctgtaactgcaaccttccactgtggttattactagtatcagaccttggtgaagcagtggccatgtcccaaaattcagctaaaactatgtatcaggaactgctagacactggggatacaaagatgagtaagacacgattccctctttcaaggagctcatagtctgtgaggagacaaccccggcgcgaagctgtcggctcccggcagccgggcggccacggcagcggcacctcctcctgcggcgggcgccctcacccttccgcgcccaagatcgccatctcgcagcaggcgcggcggcagcagccacccaggcgtcggccccggcagcccag

SEQ ID NO: 16858 - RNA, 1173 nt, Homo sapiens
  source 1..1173: mol_type = other RNA
tacgtagatatatatgtatttttagattttaatctcactagaattcatgtcttcatttttttttaagtgcccttaaaggtcatcaaatgcaagctaatacttctacctaagtctcctcatcaatcatttaatattgtttacactgcattcacagtttgtgtgttaaccacttatgtaatttatcaaatggcatatttggaaatgtaagggagaaacttggtttaggtaatactctatgtatcagttacccattacatgatttattttcatcattatttgcaacgccacacatcttgtagttttctgtgtagtctctgcatgcagtctacttcagcttctagtgctgtacatatctatatcttctgggtgggactgcccgtgatccatgagcttggggtcaggcataaactgggttgcacctgaagtggattctgatttggtctttgcttcagagctgagttctgttggcaagggcactgagtgtttcaagacgtgagttgtttttgcaggtacttctatttcggaagaggatcctagcttagttttttctttaggtttagggagtgactcttctttgctgctttttgtccacaatgatttaactgctccaaaaatttgctggcttgtagcatataccttttttgctgttaccttagcaattattacggactgaactgggtagcaaacagttgctcctaaagtggccagtcccagaggataagtaattttcttaaacttggaaccttttctcgctgaaaccaagcccgccaatcctgaaactgtaataactcccattttcggaagaaaatctcgaggaggattcttcagatagacataagcatcttttccaaattgtactgtatccattatcccatttttcacaaagacataaacacccttgcaccagccaatgtaacaaccagttgcagtgcggatggaagcaaagcccatttgtaaatgaccaggctgctcttcaacatatttagactggagcggtggtgcagtatatatggggagctgctctggtttcactagctgctttttggattcctcttgtttggctgcatgtacacttacagatgcatatatcagacctgcaggcatggttgtcagttttcccatcctgatggccgccatgtctacaaccctttcggccaaggttttcagacggag

SEQ ID NO: 16859 - RNA, 260 nt, Homo sapiens
  source 1..260: mol_type = other RNA
tacgtagatatatatgtatttttgaaaaactgctagtcacggccgagtcattttgggttccaccccttcctgcaatcaaagccttccacacgctacaaaggatttcccttataaggtaaaagaggcttgctagatacatgtggcaaaggaacaggaagatgtcagttaatcacacaaaaatctaaacgaaaccagctgtcgggaaacaggcccagaagtctaccacacgccggctcctggcttattctacaagagtgaaa

SEQ ID NO: 16860 - RNA, 5468 nt, Homo sapiens
  source 1..5468: mol_type = other RNA
tacgtagatatatatgtatttttttacacgtaaatacttgaccacttggaacttcccttagtataaaaaggagtctaatccaacttttctcttttcaaggtggcccaaacttctgagcatgggtagttgttgcaaagttccagttcctgatcacacacggcccctttgtgccacgccgagttcctgtgtatttggcttatttgtggactttcttgttccaggaatctttttaaagggccagcatcatgctgtttcaattacaatgttctaaaaacagcagaatttaaaacaatttgactagtctggcatatttgcttttctgttttaactttagaatccgcttgtgttttaaaggaaggttttacatcttaagatactgtatagcaaaatgtgagaatcaacagaactttcacttattcagggcctgtgttccttagtaatgttataatacctttcacataggtgtttccctatttgttactaggtattttatcttttttgggggttgctattgaaaaaatgacttctggtcaggtgcagtgtctcatgcctgtaatcccagcatttggggaggctgaggtaggaggttcgcttgaggccaggagtacaagaacagccttggcaacatagcaagacactgcctctataaaaaatacaataaaaattatctgggcgtggtgatgtacacctgtaggcccagctactcaggtggctgagaagagaggatcgcttgagcccagaaggtagaggctgccgtgaaacatgatcatgccactgcactccagtccaggtgacagttaagaccctgtctctaaataaaaataaaaaatgaccctccattatagcctatatttataggaaagctactgatgtttttgttaattttgtgtctggttaacttggtgaattctttcttcagtcacagattttcatttgctccttagatgacctgggtatgcaaccatctaacctgcaagtaatttcaccttctcctttccacttttacagcatttctgtctaagtgctgtttctttttcaatgatttcttctatactatttgttttaccacactgacctttaacaataaaacattaaatattgctaaataagagaatagatataaatagattttcctttcttttataaaacagaaacaggcaggccgggcatggtggctcacgcctgtaatcccagcactttgggaggccaaggcgggcagatcacctgaggttaggagttcaagaccagtctggccaacatagtgaaaccccgtctctacaaaaatacaaatattagctgggcatgatggcgggtgcctgtaatcccagctacttgggagactgaggtgggagaactgcttgaacccaggaggcggagggtgcagtgagctgagattgcaccactgcactccagcttgggcaacagagcaagactccacctcaattaaaaataaataaactaaaatggaaacaggatctccctatggtgctcaggatggtctggaactcaggctcaaacgatcctcccaccttgccctcccatagctgggactacaggcgtgagccactgtgctcaaatgaaacaaaggcacagcacaacgaatcgtccaagtaaaaaagacccacttgtcactacctggccccactggtattttgtggtagaggtggccaggaaagaataatcacttgagaggggacaggtgctccctgctctgacttctgtctagtgcactagtagtcaaagctgctaaagagttatgaagaatgtgtcatttgcatatcacaaagttttattaatgtaattttaaggccaattaaactaattttattcaaagtaagtctacattaaattacaatattaacaatctctagacacaacgaacttataagaaaaaaaaaatagaaatctgtttggtctttcttagaccacatatcatggaactcataaatgaaaattttcaaagatagaaatgacaattaaagagtgaggattttaatatggaaacccacaaggtgtcatatttcaaacccgcatgtttcaaaaagagactcttaataatttagcacaaaatcaaattatataaacttggtatattccagaaaatattgctttaaacacttatgccatgatcaaaattcctttggtagcttttaatcaaaatgaaacatgctattatgtaaaatataaagtacttttaaatgttatctcaaaagtatctttgtcatagttacccttctaacatcactactgaactttcctttcactgttcaacctcatgtatatatacacaacacaaaaccaggtaccaacaaaatccttttaatctttccacaaaataacctctgcttcacaacatcaagactttaagtctccataaactttttacagtttacagcagagaacaaggatcgtccctgcgcatgactgtaaaaaccaaaccaaactttattattgcaatcacacaaatactgcaattaaaaaaaatcaaagagcagttaccccaatgcaaaaaaacagggactgccagactcaatcttagaatggaaacacaaacacactagccccaaaccctaaaacagagattcacaaggaactcagctgacgaacagacgcagcagggcggacaccatggccttggcacctcagggagctcacttagaaacctgacttacgaaaaatcagccatcaaagtttacaacttttggaaatacatgaaacagagaggggccagtggctagggtgcgtcatccattcgccagctttgaaccctggctctttctaatgttcacccatgaagggcccttgttttcactctaaatgctgatcatctgagcgagctgtcttcagggatacctaaggaatcttcagagctaaaaaatgcagcatctagggtcttcttcattgtgcactcatgatcacacacgagaacaaaccaaacttgcagctttttgacacaagaacaagaccttttaaaggaacttctctttagtaacatcttcttgtccaatctcaaagttattttgcacagagtaacagaaacaatttaaatgcctaaaagaactagaggaaaaactggagggaaaaagatacatctgcaggttgaagtcttgagccttgtgaaagatgacccaggagccacctcccttccttcgccttccaatgtccacagctggatcaatcagagtcccagaaatggcacaggtgtgcttcctgctctgagggtacattctagtgtttcatgaaggggaaccgtctgcagatgcgtcaggccacgtagtggtactgattcggattgtctttgtctctctccatatagtctctgtctatcagagattcaattctctttttcaaatctccaggctttactggaaatttcagctgattatataattcagaaactagaagattatgaccaagagtctttctcatcttcattattctgacgatagcagcatcaatctgatattgtctatcctgaaacactctctcagtggtgctaacctgttcctcaacagtttccttcatctgaatttgattgatctttattctaaacaacttgtgcttgaactctccattaaaaatgaacttgtctccatcttccacttcctttcctttgggacttttaatcagcacacgtgctttgccacaggccagggactgcagcgttctgcgcaattcactatcctctatccccgtggccatttttatctcctcaaagctgaagccatctccctcgttgaacatgaggagcaccagtgtctggaagagggacacctggaattccttcttcccttctttaaactccgcttttaaaacagcatgtcccaaagtagtttgccactgaagttttcgaccactgtgctttccaagataaaatgccttaaatacttcctgaagtttaatcatttctggggttaagtgcacttccatgggcgtgtatgttggccagtagcccattgtgagtatgttcactgtgaggtctatagggcctgagtcactctgattctgcatatgctgcttgaaatgaaccatgatgtccttcgaaagctccatgtccttgaacatgccttccagcttgctggtgaaggctgcaccgcactcatgcttgagctttgacaacatagacttttcagcatcgactgaggcacttttcccaacaaggagtctttttgccaaatcttttttataaaatgcttcaaagacatctttaccgtggataaacctgaacaggatcatgatcttgtccaacgtccgctccagctcctcgtctgtggcttctttgttgcctgctcttaactttgaatccacatgctttgcgatcagttctgcaggcttgttgggtctcttgttgatgaacgtctcaaaggactccttcatcaggttgacgaaccgctcattcttctggaagcagacctcgatcacgtggtccaccttgtccttgaagtccaacaggtcttggaccatgtctttgtctttctcaggattgattacgatcgctgttccaaaagtcttgatgtactcgctccagtgctgcagcagcgcctgctgcccgcccctcacccggctgaacagctggtacatctgtgcgaggtccggcactctgttctcatccagtaagtggtcgagccctttctgcagaattgctgttaaatgttctcctaatagctgtttctccacacaagcaatcagtggtttctgtgtgctgtggtccaagtaagtgattactctgtctccctcttcctctaagcgtttacttacatggttaagatattctggaacctctctttcctgcattaacctttggccttcggcagcatataagcaattagtctcttccaaaaatttcagttcaaatgaatctttatacacctgcaggtcagacagcatgcccaggaggctccgcaacaggctccggtccacggcctcgccgctcctctcgcgctcgatcagcagtaggattccatcaatggttttactctgaaccattttatcactaataatatgggttctaaacagttctaatcccatatcccagatggagggcagcgtggagttctgcagcacataggtgcggtccaagaacaggaagatgcttctgatcatgatcatttgtctgcagtggtcctgccagcacgtgttaatcttctttaaaaataaaacactatctagtgagtcttctctaaacggaaggatctgtgcctggacgtggtcttcacaggcctgacgcagttgcttgtagagcattggggagactttgtgagaacagagattttccacagcctgatggaggtgctgctctgcacggcccgcaccgcctcgtgcagcttccgccacgtgtcctgcgtgtagttgtcgggcagccgaggtctgtaatcagagccgctggcgtcccggctgagaggacggggccccggcagaaagaccccgggccccctcagcccgagcgcgtcgccgagccggtccccagg

SEQ ID NO: 16861 - RNA, 5534 nt, Homo sapiens
  source 1..5534: mol_type = other RNA
tacgtagatatatatgtatttttttacacgtaaatacttgaccacttggaacttcccttagtataaaaaggagtctaatccaacttttctcttttcaaggtggcccaaacttctgagcatgggtagttgttgcaaagttccagttcctgatcacacacggcccctttgtgccacgccgagttcctgtgtatttggcttatttgtggactttcttgttccaggaatctttttaaagggccagcatcatgctgtttcaattacaatgttctaaaaacagcagaatttaaaacaatttgactagtctggcatatttgcttttctgttttaactttagaatccgcttgtgttttaaaggaaggttttacatcttaagatactgtatagcaaaatgtgagaatcaacagaactttcacttattcagggcctgtgttccttagtaatgttataatacctttcacataggtgtttccctatttgttactaggtattttatcttttttgggggttgctattgaaaaaatgacttctggtcaggtgcagtgtctcatgcctgtaatcccagcatttggggaggctgaggtaggaggttcgcttgaggccaggagtacaagaacagccttggcaacatagcaagacactgcctctataaaaaatacaataaaaattatctgggcgtggtgatgtacacctgtaggcccagctactcaggtggctgagaagagaggatcgcttgagcccagaaggtagaggctgccgtgaaacatgatcatgccactgcactccagtccaggtgacagttaagaccctgtctctaaataaaaataaaaaatgaccctccattatagcctatatttataggaaagctactgatgtttttgttaattttgtgtctggttaacttggtgaattctttcttcagtcacagattttcatttgctccttagatgacctgggtatgcaaccatctaacctgcaagtaatttcaccttctcctttccacttttacagcatttctgtctaagtgctgtttctttttcaatgatttcttctatactatttgttttaccacactgacctttaacaataaaacattaaatattgctaaataagagaatagatataaatagattttcctttcttttataaaacagaaacaggcaggccgggcatggtggctcacgcctgtaatcccagcactttgggaggccaaggcgggcagatcacctgaggttaggagttcaagaccagtctggccaacatagtgaaaccccgtctctacaaaaatacaaatattagctgggcatgatggcgggtgcctgtaatcccagctacttgggagactgaggtgggagaactgcttgaacccaggaggcggagggtgcagtgagctgagattgcaccactgcactccagcttgggcaacagagcaagactccacctcaattaaaaataaataaactaaaatggaaacaggatctccctatggtgctcaggatggtctggaactcaggctcaaacgatcctcccaccttgccctcccatagctgggactacaggcgtgagccactgtgctcaaatgaaacaaaggcacagcacaacgaatcgtccaagtaaaaaagacccacttgtcactacctggccccactggtattttgtggtagaggtggccaggaaagaataatcacttgagaggggacaggtgctccctgctctgacttctgtctagtgcactagtagtcaaagctgctaaagagttatgaagaatgtgtcatttgcatatcacaaagttttattaatgtaattttaaggccaattaaactaattttattcaaagtaagtctacattaaattacaatattaacaatctctagacacaacgaacttataagaaaaaaaaaatagaaatctgtttggtctttcttagaccacatatcatggaactcataaatgaaaattttcaaagatagaaatgacaattaaagagtgaggattttaatatggaaacccacaaggtgtcatatttcaaacccgcatgtttcaaaaagagactcttaataatttagcacaaaatcaaattatataaacttggtatattccagaaaatattgctttaaacacttatgccatgatcaaaattcctttggtagcttttaatcaaaatgaaacatgctattatgtaaaatataaagtacttttaaatgttatctcaaaagtatctttgtcatagttacccttctaacatcactactgaactttcctttcactgttcaacctcatgtatatatacacaacacaaaaccaggtaccaacaaaatccttttaatctttccacaaaataacctctgcttcacaacatcaagactttaagtctccataaactttttacagtttacagcagagaacaaggatcgtccctgcgcatgactgtaaaaaccaaaccaaactttattattgcaatcacacaaatactgcaattaaaaaaaatcaaagagcagttaccccaatgcaaaaaaacagggactgccagactcaatcttagaatggaaacacaaacacactagccccaaaccctaaaacagagattcacaaggaactcagctgacgaacagacgcagcagggcggacaccatggccttggcacctcagggagctcacttagaaacctgacttacgaaaaatcagccatcaaagtttacaacttttggaaatacatgaaacagagaggggccagtggctagggtgcgtcatccattcgccagctttgaaccctggctctttctaatgttcacccatgaagggcccttgttttcactctaaatgctgatcatctgagcgagctgtcttcagggatacctaaggaatcttcagagctaaaaaatgcagcatctagggtcttcttcattgtgcactcatgatcacacacgagaacaaaccaaacttgcagctttttgacacaagaacaagaccttttaaaggaacttctctttagtaacatcttcttgtccaatctcaaagttattttgcacagagtaacagaaacaatttaaatgcctaaaagaactagaggaaaaactggagggaaaaagatacatctgcaggttgaagtcttgagccttgtgaaagatgacccaggagccacctcccttccttcgccttccaatgtccacagctggatcaatcagagtcccagaaatggcacaggtgtgcttcctgctctgagggtacattctagtgtttcatgaaggggaaccgtctgcagatgcgtcaggccacgtagtggtactgattcggattgtctttgtctctctccatatagtctctgtctatcagagattcaattctctttttcaaatctccaggctttactggaaatttcagctgattatataattcagaaactagaagattatgaccaagagtctttctcatcttcattattctgacgatagcagcatcaatctgatattgtctatcctgaaacactctctcagtggtgctaacctgttcctcaacagtttccttcatctgaatttgattgatctttattctaaacaacttgtgcttgaactctccattaaaaatgaacttgtctccatcttccacttcctttcctttgggacttttaatcagcacacgtgctttgccacaggccagggactgcagcgttctgcgcaattcactatcctctatccccgtggccatttttatctcctcaaagctgaagccatctccctcgttgaacatgaggagcaccagtgtctggaagagggacacctggaattccttcttcccttctttaaactccgcttttaaaacagcatgtcccaaagtagtttgccactgaagttttcgaccactgtgctttccaagataaaatgccttaaatacttcctgaagtttaatcatttctggggttaagtgcacttccatgggcgtgtatgttggccagtagcccattgtgagtatgttcactgtgaggtctatagggcctgagtcactctgattctgcatatgctgcttgaaatgaaccatgatgtccttcgaaagctccatgtccttgaacatgccttccagcttgctggtgaaggctgcaccgcactcatgcttgagctttgacaacatagacttttcagcatcgactgaggcacttttcccaacaaggagtctttttgccaaatcttttttataaaatgcttcaaagacatctttaccgtggataaacctgaacaggatcatgatcttgtccaacgtccgctccagctcctcgtctgtggcttctttgttgcctgctcttaactttgaatccacatgctttgcgatcagttctgcaggcttgttgggtctcttgttgatgaacgtctcaaaggactccttcatcaggttgacgaaccgctcattcttctggaagcagacctcgatcacgtggtccaccttgtccttgaagtccaacaggtcttggaccatgtctttgtctttctcaggattgattacgatcgctgttccaaaagtcttgatgtactcgctccagtgctgcagcagcgcctgctgcccgcccctcacccggctgaacagctggtacatctgtgcgaggtccggcactctgttctcatccagtaagtggtcgagccctttctgcagaattgctgttaaatgttctcctaatagctgtttctccacacaagcaatcagtggtttctgtgtgctgtggtccaagtaagtgattactctgtctccctcttcctctaagcgtttacttacatggttaagatattctggaacctctctttcctgcattaacctttggccttcggcagcatataagcaattagtctcttccaaaaatttcagttcaaatgaatctttatacacctgcaggtcagacagcatgcccaggaggctccgcaacaggctccggtccacggcctcgccgctcctctcgcgctcgatcagcagtaggattccatcaatggttttactctgaaccattttatcactaataatatgggttctaaacagttctaatcccatatcccagatggagggcagcgtggagttctgcagcacataggtgcggtccaagaacaggaagatgcttctgatcatgatcatttgtctgcagtggtcctgccagcacgtgttaatcttctttaaaaataaaacactatctagtgagtcttctctaaacggaaggatctgtgcctggacgtggtcttcacaggcctgacgcagttgcttgtagagcattggggagactttgtgagaacagagattttccacagcctgatggaggtgctgctctgcacggcccgcaccgcctcgtgcagcttccgccacgtgtcctgcgtgtagttgtcgggcagccgaggtctgtctcggaagttcttgatgaccagcttcttggagccgcccgcgccccccggcttggcgggcgcggcggccagggccgcgggcttggtgaggccgttggtgcggcccacgagcgccgagaagctgcccttccgcggggcctcgtccgccatggctgggccggaacc

SEQ ID NO: 16862 - RNA, 5493 nt, Homo sapiens
  source 1..5493: mol_type = other RNA
tacgtagatatatatgtatttttttacacgtaaatacttgaccacttggaacttcccttagtataaaaaggagtctaatccaacttttctcttttcaaggtggcccaaacttctgagcatgggtagttgttgcaaagttccagttcctgatcacacacggcccctttgtgccacgccgagttcctgtgtatttggcttatttgtggactttcttgttccaggaatctttttaaagggccagcatcatgctgtttcaattacaatgttctaaaaacagcagaatttaaaacaatttgactagtctggcatatttgcttttctgttttaactttagaatccgcttgtgttttaaaggaaggttttacatcttaagatactgtatagcaaaatgtgagaatcaacagaactttcacttattcagggcctgtgttccttagtaatgttataatacctttcacataggtgtttccctatttgttactaggtattttatcttttttgggggttgctattgaaaaaatgacttctggtcaggtgcagtgtctcatgcctgtaatcccagcatttggggaggctgaggtaggaggttcgcttgaggccaggagtacaagaacagccttggcaacatagcaagacactgcctctataaaaaatacaataaaaattatctgggcgtggtgatgtacacctgtaggcccagctactcaggtggctgagaagagaggatcgcttgagcccagaaggtagaggctgccgtgaaacatgatcatgccactgcactccagtccaggtgacagttaagaccctgtctctaaataaaaataaaaaatgaccctccattatagcctatatttataggaaagctactgatgtttttgttaattttgtgtctggttaacttggtgaattctttcttcagtcacagattttcatttgctccttagatgacctgggtatgcaaccatctaacctgcaagtaatttcaccttctcctttccacttttacagcatttctgtctaagtgctgtttctttttcaatgatttcttctatactatttgttttaccacactgacctttaacaataaaacattaaatattgctaaataagagaatagatataaatagattttcctttcttttataaaacagaaacaggcaggccgggcatggtggctcacgcctgtaatcccagcactttgggaggccaaggcgggcagatcacctgaggttaggagttcaagaccagtctggccaacatagtgaaaccccgtctctacaaaaatacaaatattagctgggcatgatggcgggtgcctgtaatcccagctacttgggagactgaggtgggagaactgcttgaacccaggaggcggagggtgcagtgagctgagattgcaccactgcactccagcttgggcaacagagcaagactccacctcaattaaaaataaataaactaaaatggaaacaggatctccctatggtgctcaggatggtctggaactcaggctcaaacgatcctcccaccttgccctcccatagctgggactacaggcgtgagccactgtgctcaaatgaaacaaaggcacagcacaacgaatcgtccaagtaaaaaagacccacttgtcactacctggccccactggtattttgtggtagaggtggccaggaaagaataatcacttgagaggggacaggtgctccctgctctgacttctgtctagtgcactagtagtcaaagctgctaaagagttatgaagaatgtgtcatttgcatatcacaaagttttattaatgtaattttaaggccaattaaactaattttattcaaagtaagtctacattaaattacaatattaacaatctctagacacaacgaacttataagaaaaaaaaaatagaaatctgtttggtctttcttagaccacatatcatggaactcataaatgaaaattttcaaagatagaaatgacaattaaagagtgaggattttaatatggaaacccacaaggtgtcatatttcaaacccgcatgtttcaaaaagagactcttaataatttagcacaaaatcaaattatataaacttggtatattccagaaaatattgctttaaacacttatgccatgatcaaaattcctttggtagcttttaatcaaaatgaaacatgctattatgtaaaatataaagtacttttaaatgttatctcaaaagtatctttgtcatagttacccttctaacatcactactgaactttcctttcactgttcaacctcatgtatatatacacaacacaaaaccaggtaccaacaaaatccttttaatctttccacaaaataacctctgcttcacaacatcaagactttaagtctccataaactttttacagtttacagcagagaacaaggatcgtccctgcgcatgactgtaaaaaccaaaccaaactttattattgcaatcacacaaatactgcaattaaaaaaaatcaaagagcagttaccccaatgcaaaaaaacagggactgccagactcaatcttagaatggaaacacaaacacactagccccaaaccctaaaacagagattcacaaggaactcagctgacgaacagacgcagcagggcggacaccatggccttggcacctcagggagctcacttagaaacctgacttacgaaaaatcagccatcaaagtttacaacttttggaaatacatgaaacagagaggggccagtggctagggtgcgtcatccattcgccagctttgaaccctggctctttctaatgttcacccatgaagggcccttgttttcactctaaatgctgatcatctgagcgagctgtcttcagggatacctaaggaatcttcagagctaaaaaatgcagcatctagggtcttcttcattgtgcactcatgatcacacacgagaacaaaccaaacttgcagctttttgacacaagaacaagaccttttaaaggaacttctctttagtaacatcttcttgtccaatctcaaagttattttgcacagagtaacagaaacaatttaaatgcctaaaagaactagaggaaaaactggagggaaaaagatacatctgcaggttgaagtcttgagccttgtgaaagatgacccaggagccacctcccttccttcgccttccaatgtccacagctggatcaatcagagtcccagaaatggcacaggtgtgcttcctgctctgagggtacattctagtgtttcatgaaggggaaccgtctgcagatgcgtcaggccacgtagtggtactgattcggattgtctttgtctctctccatatagtctctgtctatcagagattcaattctctttttcaaatctccaggctttactggaaatttcagctgattatataattcagaaactagaagattatgaccaagagtctttctcatcttcattattctgacgatagcagcatcaatctgatattgtctatcctgaaacactctctcagtggtgctaacctgttcctcaacagtttccttcatctgaatttgattgatctttattctaaacaacttgtgcttgaactctccattaaaaatgaacttgtctccatcttccacttcctttcctttgggacttttaatcagcacacgtgctttgccacaggccagggactgcagcgttctgcgcaattcactatcctctatccccgtggccatttttatctcctcaaagctgaagccatctccctcgttgaacatgaggagcaccagtgtctggaagagggacacctggaattccttcttcccttctttaaactccgcttttaaaacagcatgtcccaaagtagtttgccactgaagttttcgaccactgtgctttccaagataaaatgccttaaatacttcctgaagtttaatcatttctggggttaagtgcacttccatgggcgtgtatgttggccagtagcccattgtgagtatgttcactgtgaggtctatagggcctgagtcactctgattctgcatatgctgcttgaaatgaaccatgatgtccttcgaaagctccatgtccttgaacatgccttccagcttgctggtgaaggctgcaccgcactcatgcttgagctttgacaacatagacttttcagcatcgactgaggcacttttcccaacaaggagtctttttgccaaatcttttttataaaatgcttcaaagacatctttaccgtggataaacctgaacaggatcatgatcttgtccaacgtccgctccagctcctcgtctgtggcttctttgttgcctgctcttaactttgaatccacatgctttgcgatcagttctgcaggcttgttgggtctcttgttgatgaacgtctcaaaggactccttcatcaggttgacgaaccgctcattcttctggaagcagacctcgatcacgtggtccaccttgtccttgaagtccaacaggtcttggaccatgtctttgtctttctcaggattgattacgatcgctgttccaaaagtcttgatgtactcgctccagtgctgcagcagcgcctgctgcccgcccctcacccggctgaacagctggtacatctgtgcgaggtccggcactctgttctcatccagtaagtggtcgagccctttctgcagaattgctgttaaatgttctcctaatagctgtttctccacacaagcaatcagtggtttctgtgtgctgtggtccaagtaagtgattactctgtctccctcttcctctaagcgtttacttacatggttaagatattctggaacctctctttcctgcattaacctttggccttcggcagcatataagcaattagtctcttccaaaaatttcagttcaaatgaatctttatacacctgcaggtcagacagcatgcccaggaggctccgcaacaggctccggtccacggcctcgccgctcctctcgcgctcgatcagcagtaggattccatcaatggttttactctgaaccattttatcactaataatatgggttctaaacagttctaatcccatatcccagatggagggcagcgtggagttctgcagcacataggtgcggtccaagaacaggaagatgcttctgatcatgatcatttgtctgcagtggtcctgccagcacgtgttaatcttctttaaaaataaaacactatctagtgagtcttctctaaacggaaggatctgtgcctggacgtggtcttcacaggcctgacgcagttgcttgtagagcattggggagactttgtgagaacagagattttccacagcctggtagagctcctcgaggttgtacctgatggaggtgctgctctgcacggcccgcaccgcctcgtgcagcttccgccacgtgtcctgcgtgtagttgtcgggcagccgaggtctgtaatcagagccgctggcgtcccggctgagaggacggggccccggcagaaagaccccgggccccctcagcccgagcgcgtcgccgagccggtccccagg

SEQ ID NO: 16863 - RNA, 5559 nt, Homo sapiens
  source 1..5559: mol_type = other RNA
tacgtagatatatatgtatttttttacacgtaaatacttgaccacttggaacttcccttagtataaaaaggagtctaatccaacttttctcttttcaaggtggcccaaacttctgagcatgggtagttgttgcaaagttccagttcctgatcacacacggcccctttgtgccacgccgagttcctgtgtatttggcttatttgtggactttcttgttccaggaatctttttaaagggccagcatcatgctgtttcaattacaatgttctaaaaacagcagaatttaaaacaatttgactagtctggcatatttgcttttctgttttaactttagaatccgcttgtgttttaaaggaaggttttacatcttaagatactgtatagcaaaatgtgagaatcaacagaactttcacttattcagggcctgtgttccttagtaatgttataatacctttcacataggtgtttccctatttgttactaggtattttatcttttttgggggttgctattgaaaaaatgacttctggtcaggtgcagtgtctcatgcctgtaatcccagcatttggggaggctgaggtaggaggttcgcttgaggccaggagtacaagaacagccttggcaacatagcaagacactgcctctataaaaaatacaataaaaattatctgggcgtggtgatgtacacctgtaggcccagctactcaggtggctgagaagagaggatcgcttgagcccagaaggtagaggctgccgtgaaacatgatcatgccactgcactccagtccaggtgacagttaagaccctgtctctaaataaaaataaaaaatgaccctccattatagcctatatttataggaaagctactgatgtttttgttaattttgtgtctggttaacttggtgaattctttcttcagtcacagattttcatttgctccttagatgacctgggtatgcaaccatctaacctgcaagtaatttcaccttctcctttccacttttacagcatttctgtctaagtgctgtttctttttcaatgatttcttctatactatttgttttaccacactgacctttaacaataaaacattaaatattgctaaataagagaatagatataaatagattttcctttcttttataaaacagaaacaggcaggccgggcatggtggctcacgcctgtaatcccagcactttgggaggccaaggcgggcagatcacctgaggttaggagttcaagaccagtctggccaacatagtgaaaccccgtctctacaaaaatacaaatattagctgggcatgatggcgggtgcctgtaatcccagctacttgggagactgaggtgggagaactgcttgaacccaggaggcggagggtgcagtgagctgagattgcaccactgcactccagcttgggcaacagagcaagactccacctcaattaaaaataaataaactaaaatggaaacaggatctccctatggtgctcaggatggtctggaactcaggctcaaacgatcctcccaccttgccctcccatagctgggactacaggcgtgagccactgtgctcaaatgaaacaaaggcacagcacaacgaatcgtccaagtaaaaaagacccacttgtcactacctggccccactggtattttgtggtagaggtggccaggaaagaataatcacttgagaggggacaggtgctccctgctctgacttctgtctagtgcactagtagtcaaagctgctaaagagttatgaagaatgtgtcatttgcatatcacaaagttttattaatgtaattttaaggccaattaaactaattttattcaaagtaagtctacattaaattacaatattaacaatctctagacacaacgaacttataagaaaaaaaaaatagaaatctgtttggtctttcttagaccacatatcatggaactcataaatgaaaattttcaaagatagaaatgacaattaaagagtgaggattttaatatggaaacccacaaggtgtcatatttcaaacccgcatgtttcaaaaagagactcttaataatttagcacaaaatcaaattatataaacttggtatattccagaaaatattgctttaaacacttatgccatgatcaaaattcctttggtagcttttaatcaaaatgaaacatgctattatgtaaaatataaagtacttttaaatgttatctcaaaagtatctttgtcatagttacccttctaacatcactactgaactttcctttcactgttcaacctcatgtatatatacacaacacaaaaccaggtaccaacaaaatccttttaatctttccacaaaataacctctgcttcacaacatcaagactttaagtctccataaactttttacagtttacagcagagaacaaggatcgtccctgcgcatgactgtaaaaaccaaaccaaactttattattgcaatcacacaaatactgcaattaaaaaaaatcaaagagcagttaccccaatgcaaaaaaacagggactgccagactcaatcttagaatggaaacacaaacacactagccccaaaccctaaaacagagattcacaaggaactcagctgacgaacagacgcagcagggcggacaccatggccttggcacctcagggagctcacttagaaacctgacttacgaaaaatcagccatcaaagtttacaacttttggaaatacatgaaacagagaggggccagtggctagggtgcgtcatccattcgccagctttgaaccctggctctttctaatgttcacccatgaagggcccttgttttcactctaaatgctgatcatctgagcgagctgtcttcagggatacctaaggaatcttcagagctaaaaaatgcagcatctagggtcttcttcattgtgcactcatgatcacacacgagaacaaaccaaacttgcagctttttgacacaagaacaagaccttttaaaggaacttctctttagtaacatcttcttgtccaatctcaaagttattttgcacagagtaacagaaacaatttaaatgcctaaaagaactagaggaaaaactggagggaaaaagatacatctgcaggttgaagtcttgagccttgtgaaagatgacccaggagccacctcccttccttcgccttccaatgtccacagctggatcaatcagagtcccagaaatggcacaggtgtgcttcctgctctgagggtacattctagtgtttcatgaaggggaaccgtctgcagatgcgtcaggccacgtagtggtactgattcggattgtctttgtctctctccatatagtctctgtctatcagagattcaattctctttttcaaatctccaggctttactggaaatttcagctgattatataattcagaaactagaagattatgaccaagagtctttctcatcttcattattctgacgatagcagcatcaatctgatattgtctatcctgaaacactctctcagtggtgctaacctgttcctcaacagtttccttcatctgaatttgattgatctttattctaaacaacttgtgcttgaactctccattaaaaatgaacttgtctccatcttccacttcctttcctttgggacttttaatcagcacacgtgctttgccacaggccagggactgcagcgttctgcgcaattcactatcctctatccccgtggccatttttatctcctcaaagctgaagccatctccctcgttgaacatgaggagcaccagtgtctggaagagggacacctggaattccttcttcccttctttaaactccgcttttaaaacagcatgtcccaaagtagtttgccactgaagttttcgaccactgtgctttccaagataaaatgccttaaatacttcctgaagtttaatcatttctggggttaagtgcacttccatgggcgtgtatgttggccagtagcccattgtgagtatgttcactgtgaggtctatagggcctgagtcactctgattctgcatatgctgcttgaaatgaaccatgatgtccttcgaaagctccatgtccttgaacatgccttccagcttgctggtgaaggctgcaccgcactcatgcttgagctttgacaacatagacttttcagcatcgactgaggcacttttcccaacaaggagtctttttgccaaatcttttttataaaatgcttcaaagacatctttaccgtggataaacctgaacaggatcatgatcttgtccaacgtccgctccagctcctcgtctgtggcttctttgttgcctgctcttaactttgaatccacatgctttgcgatcagttctgcaggcttgttgggtctcttgttgatgaacgtctcaaaggactccttcatcaggttgacgaaccgctcattcttctggaagcagacctcgatcacgtggtccaccttgtccttgaagtccaacaggtcttggaccatgtctttgtctttctcaggattgattacgatcgctgttccaaaagtcttgatgtactcgctccagtgctgcagcagcgcctgctgcccgcccctcacccggctgaacagctggtacatctgtgcgaggtccggcactctgttctcatccagtaagtggtcgagccctttctgcagaattgctgttaaatgttctcctaatagctgtttctccacacaagcaatcagtggtttctgtgtgctgtggtccaagtaagtgattactctgtctccctcttcctctaagcgtttacttacatggttaagatattctggaacctctctttcctgcattaacctttggccttcggcagcatataagcaattagtctcttccaaaaatttcagttcaaatgaatctttatacacctgcaggtcagacagcatgcccaggaggctccgcaacaggctccggtccacggcctcgccgctcctctcgcgctcgatcagcagtaggattccatcaatggttttactctgaaccattttatcactaataatatgggttctaaacagttctaatcccatatcccagatggagggcagcgtggagttctgcagcacataggtgcggtccaagaacaggaagatgcttctgatcatgatcatttgtctgcagtggtcctgccagcacgtgttaatcttctttaaaaataaaacactatctagtgagtcttctctaaacggaaggatctgtgcctggacgtggtcttcacaggcctgacgcagttgcttgtagagcattggggagactttgtgagaacagagattttccacagcctggtagagctcctcgaggttgtacctgatggaggtgctgctctgcacggcccgcaccgcctcgtgcagcttccgccacgtgtcctgcgtgtagttgtcgggcagccgaggtctgtctcggaagttcttgatgaccagcttcttggagccgcccgcgccccccggcttggcgggcgcggcggccagggccgcgggcttggtgaggccgttggtgcggcccacgagcgccgagaagctgcccttccgcggggcctcgtccgccatggctgggccggaacc

SEQ ID NO: 16864 - RNA, 5811 nt, Homo sapiens
  source 1..5811: mol_type = other RNA
tacgtagatatatatgtatttttttacacgtaaatacttgaccacttggaacttcccttagtataaaaaggagtctaatccaacttttctcttttcaaggtggcccaaacttctgagcatgggtagttgttgcaaagttccagttcctgatcacacacggcccctttgtgccacgccgagttcctgtgtatttggcttatttgtggactttcttgttccaggaatctttttaaagggccagcatcatgctgtttcaattacaatgttctaaaaacagcagaatttaaaacaatttgactagtctggcatatttgcttttctgttttaactttagaatccgcttgtgttttaaaggaaggttttacatcttaagatactgtatagcaaaatgtgagaatcaacagaactttcacttattcagggcctgtgttccttagtaatgttataatacctttcacataggtgtttccctatttgttactaggtattttatcttttttgggggttgctattgaaaaaatgacttctggtcaggtgcagtgtctcatgcctgtaatcccagcatttggggaggctgaggtaggaggttcgcttgaggccaggagtacaagaacagccttggcaacatagcaagacactgcctctataaaaaatacaataaaaattatctgggcgtggtgatgtacacctgtaggcccagctactcaggtggctgagaagagaggatcgcttgagcccagaaggtagaggctgccgtgaaacatgatcatgccactgcactccagtccaggtgacagttaagaccctgtctctaaataaaaataaaaaatgaccctccattatagcctatatttataggaaagctactgatgtttttgttaattttgtgtctggttaacttggtgaattctttcttcagtcacagattttcatttgctccttagatgacctgggtatgcaaccatctaacctgcaagtaatttcaccttctcctttccacttttacagcatttctgtctaagtgctgtttctttttcaatgatttcttctatactatttgttttaccacactgacctttaacaataaaacattaaatattgctaaataagagaatagatataaatagattttcctttcttttataaaacagaaacaggcaggccgggcatggtggctcacgcctgtaatcccagcactttgggaggccaaggcgggcagatcacctgaggttaggagttcaagaccagtctggccaacatagtgaaaccccgtctctacaaaaatacaaatattagctgggcatgatggcgggtgcctgtaatcccagctacttgggagactgaggtgggagaactgcttgaacccaggaggcggagggtgcagtgagctgagattgcaccactgcactccagcttgggcaacagagcaagactccacctcaattaaaaataaataaactaaaatggaaacaggatctccctatggtgctcaggatggtctggaactcaggctcaaacgatcctcccaccttgccctcccatagctgggactacaggcgtgagccactgtgctcaaatgaaacaaaggcacagcacaacgaatcgtccaagtaaaaaagacccacttgtcactacctggccccactggtattttgtggtagaggtggccaggaaagaataatcacttgagaggggacaggtgctccctgctctgacttctgtctagtgcactagtagtcaaagctgctaaagagttatgaagaatgtgtcatttgcatatcacaaagttttattaatgtaattttaaggccaattaaactaattttattcaaagtaagtctacattaaattacaatattaacaatctctagacacaacgaacttataagaaaaaaaaaatagaaatctgtttggtctttcttagaccacatatcatggaactcataaatgaaaattttcaaagatagaaatgacaattaaagagtgaggattttaatatggaaacccacaaggtgtcatatttcaaacccgcatgtttcaaaaagagactcttaataatttagcacaaaatcaaattatataaacttggtatattccagaaaatattgctttaaacacttatgccatgatcaaaattcctttggtagcttttaatcaaaatgaaacatgctattatgtaaaatataaagtacttttaaatgttatctcaaaagtatctttgtcatagttacccttctaacatcactactgaactttcctttcactgttcaacctcatgtatatatacacaacacaaaaccaggtaccaacaaaatccttttaatctttccacaaaataacctctgcttcacaacatcaagactttaagtctccataaactttttacagtttacagcagagaacaaggatcgtccctgcgcatgactgtaaaaaccaaaccaaactttattattgcaatcacacaaatactgcaattaaaaaaaatcaaagagcagttaccccaatgcaaaaaaacagggactgccagactcaatcttagaatggaaacacaaacacactagccccaaaccctaaaacagagattcacaaggaactcagctgacgaacagacgcagcagggcggacaccatggccttggcacctcagggagctcacttagaaacctgacttacgaaaaatcagccatcaaagtttacaacttttggaaatacatgaaacagagaggggccagtggctagggtgcgtcatccattcgccagctttgaaccctggctctttctaatgttcacccatgaagggcccttgttttcactctaaatgctgatcatctgagcgagctgtcttcagggatacctaaggaatcttcagagctaaaaaatgcagcatctagggtcttcttcattgtgcactcatgatcacacacgagaacaaaccaaacttgcagctttttgacacaagaacaagaccttttaaaggaacttctctttagtaacatcttcttgtccaatctcaaagttattttgcacagagtaacagaaacaatttaaatgcctaaaagaactagaggaaaaactggagggaaaaagatacatctgcaggttgaagtcttgagccttgtgaaagatgacccaggagccacctcccttccttcgccttccaatgtccacagctggatcaatcagagtcccagaaatggcacaggtgtgcttcctgctctgagggtacattctagtgtttcatgaaggggaaccgtctgcagatgcgtcaggccacgtagtggtactgattcggattgtctttgtctctctccatatagtctctgtctatcagagattcaattctctttttcaaatctccaggctttactggaaatttcagctgattatataattcagaaactagaagattatgaccaagagtctttctcatcttcattattctgacgatagcagcatcaatctgatattgtctatcctgaaacactctctcagtggtgctaacctgttcctcaacagtttccttcatctgaatttgattgatctttattctaaacaacttgtgcttgaactctccattaaaaatgaacttgtctccatcttccacttcctttcctttgggacttttaatcagcacacgtgctttgccacaggccagggactgcagcgttctgcgcaattcactatcctctatccccgtggccatttttatctcctcaaagctgaagccatctccctcgttgaacatgaggagcaccagtgtctggaagagggacacctggaattccttcttcccttctttaaactccgcttttaaaacagcatgtcccaaagtagtttgccactgaagttttcgaccactgtgctttccaagataaaatgccttaaatacttcctgaagtttaatcatttctggggttaagtgcacttccatgggcgtgtatgttggccagtagcccattgtgagtatgttcactgtgaggtctatagggcctgagtcactctgattctgcatatgctgcttgaaatgaaccatgatgtccttcgaaagctccatgtccttgaacatgccttccagcttgctggtgaaggctgcaccgcactcatgcttgagctttgacaacatagacttttcagcatcgactgaggcacttttcccaacaaggagtctttttgccaaatcttttttataaaatgcttcaaagacatctttaccgtggataaacctgaacaggatcatgatcttgtccaacgtccgctccagctcctcgtctgtggcttctttgttgcctgctcttaactttgaatccacatgctttgcgatcagttctgcaggcttgttgggtctcttgttgatgaacgtctcaaaggactccttcatcaggttgacgaaccgctcattcttctggaagcagacctcgatcacgtggtccaccttgtccttgaagtccaacaggtcttggaccatgtctttgtctttctcaggattgattacgatcgctgttccaaaagtcttgatgtactcgctccagtgctgcagcagcgcctgctgcccgcccctcacccggctgaacagctggtacatctgtgcgaggtccggcactctgttctcatccagtaagtggtcgagccctttctgcagaattgctgttaaatgttctcctaatagctgtttctccacacaagcaatcagtggtttctgtgtgctgtggtccaagtaagtgattactctgtctccctcttcctctaagcgtttacttacatggttaagatattctggaacctctctttcctgcattaacctttggccttcggcagcatataagcaattagtctcttccaaaaatttcagttcaaatgaatctttatacacctgcaggtcagacagcatgcccaggaggctccgcaacaggctccggtccacggcctcgccgctcctctcgcgctcgatcagcagtaggattccatcaatggttttactctgaaccattttatcactaataatatgggttctaaacagttctaatcccatatcccagatggagggcagcgtggagttctgcagcacataggtgcggtccaagaacaggaagatgcttctgatcatgatcatttgtctgcagtggtcctgccagcacgtgttaatcttctttaaaaataaaacactatctagtgagtcttctctaaacggaaggatctgtgcctggacgtggtcttcacaggcctgacgcagttgcttgtagagcattggggagactttgtgagaacagagattttccacagcctggtagagctcctcgaggttgtacctgatggaggtgctgctctgcacggcccgcaccgcctcgtgcagcttccgccacgtgtcctgcgtgtagttgtcgggcagccgaggtctgtctgcagcaggtgggtcctagccggggagcgcgcggcggcgtggttggccctcggcgtgttccgtgtgtcccctcctgccttggaccctcaggccttttcctttcccgcctcgccacccttcttccgttcgggtccccggcgggcagccgcgcgagccgaacagcggcggccgggactcgggaaggcggcccgagttctcccctgcagggccgccgtgggggccgggcggtgtccgtggatcgcggagtcgtcgcggtgtaagtagacgcggcggtcccaggtcgctgccctcacttgctggcacgtgtggccgcgctcccaggcggtccgaagggcctgcgggccacgccgagggcccgctgtgggcggtgctgtgtcggatggacgctgtttcccagcaggatgcgggatgaat

SEQ ID NO: 16865 - RNA, 5455 nt, Homo sapiens
  source 1..5455: mol_type = other RNA
tacgtagatatatatgtatttttttacacgtaaatacttgaccacttggaacttcccttagtataaaaaggagtctaatccaacttttctcttttcaaggtggcccaaacttctgagcatgggtagttgttgcaaagttccagttcctgatcacacacggcccctttgtgccacgccgagttcctgtgtatttggcttatttgtggactttcttgttccaggaatctttttaaagggccagcatcatgctgtttcaattacaatgttctaaaaacagcagaatttaaaacaatttgactagtctggcatatttgcttttctgttttaactttagaatccgcttgtgttttaaaggaaggttttacatcttaagatactgtatagcaaaatgtgagaatcaacagaactttcacttattcagggcctgtgttccttagtaatgttataatacctttcacataggtgtttccctatttgttactaggtattttatcttttttgggggttgctattgaaaaaatgacttctggtcaggtgcagtgtctcatgcctgtaatcccagcatttggggaggctgaggtaggaggttcgcttgaggccaggagtacaagaacagccttggcaacatagcaagacactgcctctataaaaaatacaataaaaattatctgggcgtggtgatgtacacctgtaggcccagctactcaggtggctgagaagagaggatcgcttgagcccagaaggtagaggctgccgtgaaacatgatcatgccactgcactccagtccaggtgacagttaagaccctgtctctaaataaaaataaaaaatgaccctccattatagcctatatttataggaaagctactgatgtttttgttaattttgtgtctggttaacttggtgaattctttcttcagtcacagattttcatttgctccttagatgacctgggtatgcaaccatctaacctgcaagtaatttcaccttctcctttccacttttacagcatttctgtctaagtgctgtttctttttcaatgatttcttctatactatttgttttaccacactgacctttaacaataaaacattaaatattgctaaataagagaatagatataaatagattttcctttcttttataaaacagaaacaggcaggccgggcatggtggctcacgcctgtaatcccagcactttgggaggccaaggcgggcagatcacctgaggttaggagttcaagaccagtctggccaacatagtgaaaccccgtctctacaaaaatacaaatattagctgggcatgatggcgggtgcctgtaatcccagctacttgggagactgaggtgggagaactgcttgaacccaggaggcggagggtgcagtgagctgagattgcaccactgcactccagcttgggcaacagagcaagactccacctcaattaaaaataaataaactaaaatggaaacaggatctccctatggtgctcaggatggtctggaactcaggctcaaacgatcctcccaccttgccctcccatagctgggactacaggcgtgagccactgtgctcaaatgaaacaaaggcacagcacaacgaatcgtccaagtaaaaaagacccacttgtcactacctggccccactggtattttgtggtagaggtggccaggaaagaataatcacttgagaggggacaggtgctccctgctctgacttctgtctagtgcactagtagtcaaagctgctaaagagttatgaagaatgtgtcatttgcatatcacaaagttttattaatgtaattttaaggccaattaaactaattttattcaaagtaagtctacattaaattacaatattaacaatctctagacacaacgaacttataagaaaaaaaaaatagaaatctgtttggtctttcttagaccacatatcatggaactcataaatgaaaattttcaaagatagaaatgacaattaaagagtgaggattttaatatggaaacccacaaggtgtcatatttcaaacccgcatgtttcaaaaagagactcttaataatttagcacaaaatcaaattatataaacttggtatattccagaaaatattgctttaaacacttatgccatgatcaaaattcctttggtagcttttaatcaaaatgaaacatgctattatgtaaaatataaagtacttttaaatgttatctcaaaagtatctttgtcatagttacccttctaacatcactactgaactttcctttcactgttcaacctcatgtatatatacacaacacaaaaccaggtaccaacaaaatccttttaatctttccacaaaataacctctgcttcacaacatcaagactttaagtctccataaactttttacagtttacagcagagaacaaggatcgtccctgcgcatgactgtaaaaaccaaaccaaactttattattgcaatcacacaaatactgcaattaaaaaaaatcaaagagcagttaccccaatgcaaaaaaacagggactgccagactcaatcttagaatggaaacacaaacacactagccccaaaccctaaaacagagattcacaaggaactcagctgacgaacagacgcagcagggcggacaccatggccttggcacctcagggagctcacttagaaacctgacttacgaaaaatcagccatcaaagtttacaacttttggaaatacatgaaacagagaggggccagtggctagggtgcgtcatccattcgccagctttgaaccctggctctttctaatgttcacccatgaagggcccttgttttcactctaaatgctgatcatctgagcgagctgtcttcagggatacctaaggaatcttcagagctaaaaaatgcagcatctagggtcttcttcattgtgcactcatgatcacacacgagaacaaaccaaacttgcagctttttgacacaagaacaagaccttttaaaggaacttctctttagtaacatcttcttgtccaatctcaaagttattttgcacagagtaacagaaacaatttaaatgcctaaaagaactagaggaaaaactggagggaaaaagatacatctgcaggttgaagtcttgagccttgtgaaagatgacccaggagccacctcccttccttcgccttccaatgtccacagctggatcaatcagagtcccagaaatggcacaggtgtgcttcctgctctgagggtacattctagtgtttcatgaaggggaaccgtctgcagatgcgtcaggccacgtagtggtactgattcggattgtctttgtctctctccatatagtctctgtctatcagagattcaattctctttttcaaatctccaggctttactggaaatttcagctgattatataattcagaaactagaagattatgaccaagagtctttctcatcttcattattctgacgatagcagcatcaatctgatattgtctatcctgaaacactctctcagtggtgctaacctgttcctcaacagtttccttcatctgaatttgattgatctttattctaaacaacttgtgcttgaactctccattaaaaatgaacttgtctccatcttccacttcctttcctttgggacttttaatcagcacacgtgctttgccacaggccagggactgcagcgttctgcgcaattcactatcctctatccccgtggccatttttatctcctcaaagctgaagccatctccctcgttgaacatgaggagcaccagtgtctggaagagggacacctggaattccttcttcccttctttaaactccgcttttaaaacagcatgtcccaaagtagtttgccactgaagttttcgaccactgtgctttccaagataaaatgccttaaatacttcctgaagtttaatcatttctggggttaagtgcacttccatgggcgtgtatgttggccagtagcccattgtgagtatgttcactgtgaggtctatagggcctgagtcactctgattctgcatatgctgcttgaaatgaaccatgatgtccttcgaaagctccatgtccttgaacatgccttccagcttgctggtgaaggctgcaccgcactcatgcttgagctttgacaacatagacttttcagcatcgactgaggcacttttcccaacaaggagtctttttgccaaatcttttttataaaatgcttcaaagacatctttaccgtggataaacctgaacaggatcatgatcttgtccaacgtccgctccagctcctcgtctgtggcttctttgttgcctgctcttaactttgaatccacatgctttgcgatcagttctgcaggcttgttgggtctcttgttgatgaacgtctcaaaggactccttcatcaggttgacgaaccgctcattcttctggaagcagacctcgatcacgtggtccaccttgtccttgaagtccaacaggtcttggaccatgtctttgtctttctcaggattgattacgatcgctgttccaaaagtcttgatgtactcgctccagtgctgcagcagcgcctgctgcccgcccctcacccggctgaacagctggtacatctgtgcgaggtccggcactctgttctcatccagtaagtggtcgagccctttctgcagaattgctgttaaatgttctcctaatagctgtttctccacacaagcaatcagtggtttctgtgtgctgtggtccaagtaagtgattactctgtctccctcttcctctaagcgtttacttacatggttaagatattctggaacctctctttcctgcattaacctttggccttcggcagcatataagcaattagtctcttccaaaaatttcagttcaaatgaatctttatacacctgcaggtcagacagcatgcccaggaggctccgcaacaggctccggtccacggcctcgccgctcctctcgcgctcgatcagcagtaggattccatcaatggttttactctgaaccattttatcactaataatatgggttctaaacagttctaatcccatatcccagatggagggcagcgtggagttctgcagcacataggtgcggtccaagaacaggaagatgcttctgatcatgatcatttgtctgcagtggtcctgccagcacgtgttaatcttctttaaaaataaaacactatctagtgagtcttctctaaacggaaggatctgtgcctggacgtggtcttcacaggcctgacgcagttgcttgtagagcattggggagactttgtgagaacagagattttccacagcctggtagagctcctcgaggttgtacctgatggaggtgctgctctgcacggcccgcaccgcctcgtgcagcttccgccacgtgtcctgcgtgtagttgtcgggcagccgaggtctgtctgcgcacccgcggcggggccgggggcgccaggacccagacggaccgagggccggaagt

SEQ ID NO: 16866 - RNA, 5557 nt, Homo sapiens
  source 1..5557: mol_type = other RNA
tacgtagatatatatgtatttttttacacgtaaatacttgaccacttggaacttcccttagtataaaaaggagtctaatccaacttttctcttttcaaggtggcccaaacttctgagcatgggtagttgttgcaaagttccagttcctgatcacacacggcccctttgtgccacgccgagttcctgtgtatttggcttatttgtggactttcttgttccaggaatctttttaaagggccagcatcatgctgtttcaattacaatgttctaaaaacagcagaatttaaaacaatttgactagtctggcatatttgcttttctgttttaactttagaatccgcttgtgttttaaaggaaggttttacatcttaagatactgtatagcaaaatgtgagaatcaacagaactttcacttattcagggcctgtgttccttagtaatgttataatacctttcacataggtgtttccctatttgttactaggtattttatcttttttgggggttgctattgaaaaaatgacttctggtcaggtgcagtgtctcatgcctgtaatcccagcatttggggaggctgaggtaggaggttcgcttgaggccaggagtacaagaacagccttggcaacatagcaagacactgcctctataaaaaatacaataaaaattatctgggcgtggtgatgtacacctgtaggcccagctactcaggtggctgagaagagaggatcgcttgagcccagaaggtagaggctgccgtgaaacatgatcatgccactgcactccagtccaggtgacagttaagaccctgtctctaaataaaaataaaaaatgaccctccattatagcctatatttataggaaagctactgatgtttttgttaattttgtgtctggttaacttggtgaattctttcttcagtcacagattttcatttgctccttagatgacctgggtatgcaaccatctaacctgcaagtaatttcaccttctcctttccacttttacagcatttctgtctaagtgctgtttctttttcaatgatttcttctatactatttgttttaccacactgacctttaacaataaaacattaaatattgctaaataagagaatagatataaatagattttcctttcttttataaaacagaaacaggcaggccgggcatggtggctcacgcctgtaatcccagcactttgggaggccaaggcgggcagatcacctgaggttaggagttcaagaccagtctggccaacatagtgaaaccccgtctctacaaaaatacaaatattagctgggcatgatggcgggtgcctgtaatcccagctacttgggagactgaggtgggagaactgcttgaacccaggaggcggagggtgcagtgagctgagattgcaccactgcactccagcttgggcaacagagcaagactccacctcaattaaaaataaataaactaaaatggaaacaggatctccctatggtgctcaggatggtctggaactcaggctcaaacgatcctcccaccttgccctcccatagctgggactacaggcgtgagccactgtgctcaaatgaaacaaaggcacagcacaacgaatcgtccaagtaaaaaagacccacttgtcactacctggccccactggtattttgtggtagaggtggccaggaaagaataatcacttgagaggggacaggtgctccctgctctgacttctgtctagtgcactagtagtcaaagctgctaaagagttatgaagaatgtgtcatttgcatatcacaaagttttattaatgtaattttaaggccaattaaactaattttattcaaagtaagtctacattaaattacaatattaacaatctctagacacaacgaacttataagaaaaaaaaaatagaaatctgtttggtctttcttagaccacatatcatggaactcataaatgaaaattttcaaagatagaaatgacaattaaagagtgaggattttaatatggaaacccacaaggtgtcatatttcaaacccgcatgtttcaaaaagagactcttaataatttagcacaaaatcaaattatataaacttggtatattccagaaaatattgctttaaacacttatgccatgatcaaaattcctttggtagcttttaatcaaaatgaaacatgctattatgtaaaatataaagtacttttaaatgttatctcaaaagtatctttgtcatagttacccttctaacatcactactgaactttcctttcactgttcaacctcatgtatatatacacaacacaaaaccaggtaccaacaaaatccttttaatctttccacaaaataacctctgcttcacaacatcaagactttaagtctccataaactttttacagtttacagcagagaacaaggatcgtccctgcgcatgactgtaaaaaccaaaccaaactttattattgcaatcacacaaatactgcaattaaaaaaaatcaaagagcagttaccccaatgcaaaaaaacagggactgccagactcaatcttagaatggaaacacaaacacactagccccaaaccctaaaacagagattcacaaggaactcagctgacgaacagacgcagcagggcggacaccatggccttggcacctcagggagctcacttagaaacctgacttacgaaaaatcagccatcaaagtttacaacttttggaaatacatgaaacagagaggggccagtggctagggtgcgtcatccattcgccagctttgaaccctggctctttctaatgttcacccatgaagggcccttgttttcactctaaatgctgatcatctgagcgagctgtcttcagggatacctaaggaatcttcagagctaaaaaatgcagcatctagggtcttcttcattgtgcactcatgatcacacacgagaacaaaccaaacttgcagctttttgacacaagaacaagaccttttaaaggaacttctctttagtaacatcttcttgtccaatctcaaagttattttgcacagagtaacagaaacaatttaaatgcctaaaagaactagaggaaaaactggagggaaaaagatacatctgcaggttgaagtcttgagccttgtgaaagatgacccaggagccacctcccttccttcgccttccaatgtccacagctggatcaatcagagtcccagaaatggcacaggtgtgcttcctgctctgagggtacattctagtgtttcatgaaggggaaccgtctgcagatgcgtcaggccacgtagtggtactgattcggattgtctttgtctctctccatatagtctctgtctatcagagattcaattctctttttcaaatctccaggctttactggaaatttcagctgattatataattcagaaactagaagattatgaccaagagtctttctcatcttcattattctgacgatagcagcatcaatctgatattgtctatcctgaaacactctctcagtggtgctaacctgttcctcaacagtttccttcatctgaatttgattgatctttattctaaacaacttgtgcttgaactctccattaaaaatgaacttgtctccatcttccacttcctttcctttgggacttttaatcagcacacgtgctttgccacaggccagggactgcagcgttctgcgcaattcactatcctctatccccgtggccatttttatctcctcaaagctgaagccatctccctcgttgaacatgaggagcaccagtgtctggaagagggacacctggaattccttcttcccttctttaaactccgcttttaaaacagcatgtcccaaagtagtttgccactgaagttttcgaccactgtgctttccaagataaaatgccttaaatacttcctgaagtttaatcatttctggggttaagtgcacttccatgggcgtgtatgttggccagtagcccattgtgagtatgttcactgtgaggtctatagggcctgagtcactctgattctgcatatgctgcttgaaatgaaccatgatgtccttcgaaagctccatgtccttgaacatgccttccagcttgctggtgaaggctgcaccgcactcatgcttgagctttgacaacatagacttttcagcatcgactgaggcacttttcccaacaaggagtctttttgccaaatcttttttataaaatgcttcaaagacatctttaccgtggataaacctgaacaggatcatgatcttgtccaacgtccgctccagctcctcgtctgtggcttctttgttgcctgctcttaactttgaatccacatgctttgcgatcagttctgcaggcttgttgggtctcttgttgatgaacgtctcaaaggactccttcatcaggttgacgaaccgctcattcttctggaagcagacctcgatcacgtggtccaccttgtccttgaagtccaacaggtcttggaccatgtctttgtctttctcaggattgattacgatcgctgttccaaaagtcttgatgtactcgctccagtgctgcagcagcgcctgctgcccgcccctcacccggctgaacagctggtacatctgtgcgaggtccggcactctgttctcatccagtaagtggtcgagccctttctgcagaattgctgttaaatgttctcctaatagctgtttctccacacaagcaatcagtggtttctgtgtgctgtggtccaagtaagtgattactctgtctccctcttcctctaagcgtttacttacatggttaagatattctggaacctctctttcctgcattaacctttggccttcggcagcatataagcaattagtctcttccaaaaatttcagttcaaatgaatctttatacacctgcaggtcagacagcatgcccaggaggctccgcaacaggctccggtccacggcctcgccgctcctctcgcgctcgatcagcagtaggattccatcaatggttttactctgaaccattttatcactaataatatgggttctaaacagttctaatcccatatcccagatggagggcagcgtggagttctgcagcacataggtgcggtccaagaacaggaagatgcttctgatcatgatcatttgtctgcagtggtcctgccagcacgtgttaatcttctttaaaaataaaacactatctagtgagttctctaaacggaaggatctgtgcctggacgtggtcttcacaggcctgacgcagttgcttgtagagcattggggagactttgtgagaacagagattttccacagcctggtagagctcctcgaggttgtacctgatggaggtgctgctctgcacggcccgcaccgcctcgtgcagcttccgccacgtgtcctgcgtgtagttgtcgggcagccgaggtctgtctcggaagttcttgatgaccagcttcttggagccgcccgcgccccccggcttggcgggcgcggcggccagggccgcgggcttggtgaggccgttggtgcggcccacgagcgccgagaagctgcccttccgcggggcctcgtccgccatggctgggccggaacc
